European Patent Application EP 4 520 821 A1 - sequence listing, part 4

SEQ ID NO: 10736 - RNA, 11301 nt, Homo sapiens
  source 1..11301: mol_type = other RNA
ctcatctgcaaagaagtaagtgggcaacgtcaaataaagttaaacggcatacacagggctgtagcttaaaccatatgtgtgtatatataagatatttgattgaaatttatgaatttattaatgtggccaaatcacggaaacaaatacatggatctatttgggatctagttggttatatggctgataaacatatggctgataaattataaataaccaaaacattgtggtaaaagagtcaaagaaaaaatgaagtaattgtgcaaggttaatatgaacagcagaaggaatgtaaaaatgtaaagtggtcttctaattcttatgtaagctttgtcatagttattaaaaagacggtatcatattagaaagcccccacccactttcccaatgctgtatacattatacaaatccgtgacaaatgtattaccatttccaaatacctctctgttcattaatttacacttgcatagaaagggaagaagaaaacaataatatatggttattataaaaacaaaatatccatttctctttggatagtcagtgttttactctttcagtagaacacacagtcagcactcaacatcgtgggccaaggagccatggagcttctgatttaatggaacttggaattggcatttgctgaaaagggcaacactgtacgtcaggaaacattggttggccggatgaatacttcacattgcctgtggcctgctgggaacatttgggcagcaagatggaaacgtgctgtgaatctgctccatgacctccgtgagatccgtgctggtgtcgtgcggtggggccagcaggtcctctcccgctgcctggtggaactgtgggccggaggcatctggatcaagcgagtagctcagtgcagaatgctgaggagaagcccatggggaaacaccattgattcgggaatcagattcaggctgctccagcagctgtcggaggcggtggagctgagactccagctgtttattgtgatcttctaaaatctgcatcctagcctccagccgacctttgtgctgcctgaggagttttgcttctgctataagttctgaatcctcagacgtgtgatggggagatataatcgactctggcggtgaaccgacagggagcccccttcggaggtgctggtccttcagctgctcatactccacctgtagatttctttgttcttcctccaggtcagcaatgatcctctccagttctccacgttcttccctctctactgacttcaggatctgagctgggctctgcggctggctcactggggactctcctccgagtgtttggcaatactgctggatgagggcgtgctcgtcttccacacttcctgtggtggagctgctatcagtgagaaaagacccattagtcctttccatctgggccagtcgtgtggcatattgttctattcttgaatgggtgtcatcatgaaacagttgaggagattgtgaggggtcatagtgctctggccacatactgatgagtgtgataggagtctctaagttgtcaccttcaagaactgtctggacaggcaggtaaccaagtcgagggtgtttggcaaagtacttcttcgacctgaacttgttcttaagtacctttgtgaagtctcgtacatcttccccagatgttgtaggtatacaatattccaccattgggtaatgtaatttgtgaccttttgctgttcgacccgaaaagaaacaactctggcagacatcatagttaaaatgcttaaggcttctatacctgaacccgacaattggacattctttacagatgttgcatttggcctgatgttttgcagtctccgctgctgccactcgatgtaaaactgggagccaaaccatggactgtggttccaaatgcatccaatctataaactctttcacacttatttctggtttattgttattctgttggaagcagctgcgaacactaggctcaatattactgcctccaaaagctgctacttcacctagctgccgggggatctggatggcatcatgaagtaacaggcccagctgcctctggtcacacatttctgttggccctgcaacttccttaaagagatatctgtatttttcttccaagagacctttggagagagacattaatccaatcttcagactctgcactctaatttttccagttcgacccgtgtcatagacattgagcaaccaattgagacacatatcaacacagagtggaacgttgaccaggtccttatgcatttgctcaagtccatcataagttgttgtcagacagttgatgacatctggaacactgaggagctggtcattttggttcaacttgtgctgtttgaaaatttcatttgttgtactcaactctaagagatccaaacatagtgctttttgtagtcttcggattttgattgctgtacggtaggcagaaaaacgtacattattcaggtcagcaagggattgaaagagttcggtcattttaggatggtcccaacaggtggtctgtgtttgatggttgatgtaatagggcactttattatgtgaaatggatctttgccacggcagctggactgacgtagagagaaaatgctgagaggatggtccaaaatctctgtgggcttcctgaagctgtttaaggcgatcatccacagaaacctgtaaaagtttccatcgcatattaaggtcatctagctggcgagacatctttagagagggatgcaggtcaagtggagacagctgactggataaatcattcaccgttttaactttaaagttgattggtgcaatttcttctctaaatgccatgattttttcaatgtgatcctgcagcgagtcaatgagtaagtctcccacgggcttccagccattccgcacggactctgcctccttcatgtcagcgtccaggtcatccatagctccctgcaggtctctgagtttctccaatgccttgtccacttgcttttgccaattgctagttacagcatttagactttcccatttttctttgacttcagaagactgtttgcgcatggctttggcaatcttttgggctctctcctcaggagttaattctgtttttgattgtaggtttcttcttggctcttcaggggcctcaattggctgatcagccaagaaaactcgggcctggtcgacagcattcaggacagaatattctttctcctttaactcccgtctcagggccttacaatggtcatactggagctgtaaggctggaacatctcctccaataggcatttgtttcttaagctcttcatctttcatattcagccatttgatcagttcttctaaggacatcagcaacctgttccacttctcagcgctggcctccaaatgggccctgatgctagcagattttgcttttaagtcattccatctttggttcatatcatccagtcgatgttgaagcatagtagcctcttcagaatttcccaaagcttttaccatcttctgcctgtttccgtcaatgcttttaaatatgtcattgtgggcatcaatttctgcctggatgtcctgcatctgctgtttgagttccctggccaagatactatcctgaagagcattctcccgatgagaggcatccacaagcacattcactgtggtctctgcttcttggatccacttcaggaagttttccagatctctgcgagaggcctgcaccgtcctccactcagcctccaaggcgttctgtctgtcagcaatactttgtttgagattgatccatgatgtttttaagtactctgtggtttctttcacattccttgtgtcatcactcccatattcctccaggagtttctgcaggacgttatcgaacgccatgacgataccatctccaggacccagttcttgaagcagtatttggttatcagaaatttgtttggtgagtggatcccgtcgggcttgctgaagaatatagagtcgagcctcatattttctcatcagttcttcagtctcctccctatggtcatcccactgaagactgtcaataatcatgtcctcaagctgctgctgtcttagctcaacgccatgctgggtgccatcccactggttcttgaccctttccaatttttctgtaattgctgttctcatatctgaactggaagctttatttttcaaattctgtgccaatgtaaaaacataatccagctgaggatggcgctgttctaagtcagcctttgtaattttcattcgggaaacggtcttattgatctcttctacatccccaacagtgacaatgttggacttcagcatctggtcgattaataccagccagtcggctagttctgttatagttttatcaagatcagcaggaattgaaatttccgaagtacgatgagactgaacaggaatatctgacgcagatgatactagcaccaccttttggacattaggatgagcagcaatccttgtctgtgaaacagaactgggctcctggatgcattccttcagggtggtaggcacctctctgcaaatcttattccatgtcatatttacagtccttaagctttctgaaattttatccctttcaggtaaactcagacttttatctgaaagcatctccaattcagttctattcagccatttgagtttttcagcatgtacttccatttcttgagttaagtctcttaattcttgcaggttttctcccaattcggtggttgatctcttttgcatagcatgctcagcctttgttaaccaacagataatctcatctagctgatgcctgtacttcatcacctgcttactttctccttttagccttggctgcctatccttcacttctgcaacaattgcatcccagcgttggtttaaacctgccagtttttctttcaagaagcttccatctgcctgggagagtttctgcacaatcccatccccagttcggtttagtgctgcaaaactgggctggtggctgctgatgcccacctcaagttcctgctgatgtatcctggctttctctaagtccaggctgccacctggagcacaggtatcaaccagtaattcttcagcctctgttatccactgtgtgaggtcattaaggtcacaatggaactgtctccattcttccattgccctgtcaaaacaacctttccgatcactgtacattctattaattctgtcccattttgcattcagctgagtaagtgtatctctgatctgaatggcttcaggtccagaggcttcaaggatgacatctggctgtttttcatgaatgactgcaatctgctctccaagtttgtccagttggtctttgatattcttcagagagtcttcctgaaaagagaagtcttcgtaaatagcagtgttgagctctggaacattaagcgataattcaacatcatccatgcaaagtaaaattttgttaatttcaaccagataatctgtaggaagaagtgatgatctaattccagaagcaagttgacccattttcctctgttgaatagggattgccttaattttgttgtatctagtatgcaaaagtaataattgcaaacggatcttttcttttttattatcttccataggttgatgtaacatttcttctcctctttgtagaacttcctcaatctgggcactctcctcatccatcttttcatcttcatcactggattccaagtgtttttccacaaattttaacatattttctatgtcattttctaatttttccaagtcagagaaaggcacaccagtttcaaatgtttcagtggtgaccaaacattggtataatggttcctgagcaattagcaatttggcacttttgatatgttgagacaccttttcaaagttcctattcagctcagctaactttggttctacaagctccctgcttgagcttccacgggcattcatcaaaataagggcttgatcgcggacattttcaacctggaggttggcatcatccagctcagatactaaacgcttcacaatttcttcctgtttacttgttggtttcttttcaatttcatccaatagagcttcagcttgataaagccaggtacttatgtgagccacgttcccatcaaatatttctagctggttctgatggttcatcaaggtattgcaccaatcttcagtccaggtacgaactcggctccacccagcgttaaggacgcagagcctctcttctaaaataggctcactgccctcaatcaagttttgcagggcagcactactctctgtgatggtatttaaatcagcttttctcttttccagatccttcagaacatttttagcccaggaaatttctgtatccaagtcaccaagcagaccttctgaagtggacttctgtaccaattcagtttcagtagcagaaagccattcagagagagaagcagcctctttcttcattttccgggccaactgtgatgctctttccagatcctgttttccttctgtcacctgtgcgcccaggtcattgtaaagaaccttcagggaagtcagctgctcatccatcccttttgggttgtccgtttgctgtttctggacaatatgtcttcctgttttaatcacagtttccacttcaagtttgacttcactcaaagttttatacagtttcatacacttgtccaggtgcgtctgtatgacgtcagggtctacgtccttcacatccagaacgtgaagttctgctttcacgccatccagcacacgcttgcagtccagcatgcgctgctcgaagttagctggcttctggaaaagctggaactttgtggacacctctcggagtttcctctgtagcacatccatctgacttcctcctctggcagtcctactctctggggaggtcaggggctgagaacgcatatttcttctcaactcctctagggttagctcatgggctgagatctctgcttggattttctgagcttcctgtggaacttggaaagcatctatcctgtcagtcaggtatgtggtgagctgtttgtccagctcccccaagctctcttgcaagacttgaagcatctggtcagtttcccgcagcacctggagttgcttttccaaagaaatctgcttgctctctgccaggtgacttagatcttcatatcggctgttgaaagcctccagtttctcactgattatatcatccaggatccccccatcaatcagagtctggccaagctctcgaatctgggtgcgattatctgccgggtggcgcagaacagattccagagactccagggcttcgttgacagcatccgtcttctcaggcaggacctctgtgctcttcatccgctcttccaaagtgtttaaccaggtagtttcaagatccaaatagtgaagcagttcaatccaacaagaccagacctcctctagcgtgtggcactttcctcgaattctattacaaagaagttggtaattctccagcacaacattcagctcagacgtcaactcctggccaccagagggcaccttggcagctaataacttgatgttgtccttgagaatcttcactctcacctccttctgcaacacatcctcttttgccctcttcatctcttccacagcactctcaagctcttctggtgacttgtactcaaaatcccgctccaaatattcttcctcggcctgggtcatccattcctgcatctctgccaagtctttcttcaggttcgcagctttttcttgactttcagacaacctacttttttgagtagcgatctccttgctaagtttctccagttgagtttggtagtcacctagtcttgtctgcacccaagtttttattccagcaactggaccacttcgaagattagtctctatttccttcatgtttttcagagatgattcaattgtttctatttcattaacaaatgcagagcactggtctaactgcctctgtagacctgcgtcgtctccttgggcagcctgctgtttcattaagaagtctttcacgccatccatccacttctcaatgactgttgaatcggcctcaaaagctctgagtgtgagagcaatttcctcaagcaaatgtagatctttggaaaccaagacctttagcttgttccactttccttgcacatcatcaaattcttgcttatataatttttctacatcaggatgaacatttttctccagagcctttgtttcttctgcaagtttatgtaatgcaggtttctgattctcaaggatttcatcaagggtctttttttcttgcagggccttctccaccttggcaagatcattaaggacattcagagacacctgggccttattttctgaatcatttagcacatctttcagtgttttcaatgtttccagatatgcatgtccaggttggcccttcagttcattctctagatgttgttgacgatcctctacagcctcttgtacagcttggtagcggcccagaaagctatcgaagccccgctggacaaaatctggggcagaaggctgagacatcagggccgagcagcttgcacgagccatttcaattttggggtgaaggccaagaagatttgtcaattcccgctgacaggaatccttcaagcttggcaaggactgccgggaagattcagaaatggaagtgtgttttacccactcctcctttgtcttgatgaccttttcaagctcatcaagctgcttgaaataagcatttatatcttcctgtagctgaatctttctttctagatcttccaaatgttgagatacattcttccattctgatgaaaccttctccagaacattttttatttcttcagtaggaaggccttcttttcccatttgctccacaaggatttgtccagtttggtttaattcatctgctctggggattctttctctctgttctttttctaatgccttcaacttctttttcatttcggaagtgtcttgcatcttcatatactcttttatctctgtggtctgaatggcagttttccatttcaaaatccagttcaacagctctgcacttatagcatcaaactttttcttagcttcaatatccacatggatctgtctcttctttgggggaggaggaggaggcagttcctgcttagatttttttgtaattgcttgttctcttacacgaacagtctccaaaaggtccttctgaggaatctgagacatccccagctttgctacagcctgagtcacctggttggaggaatcttctagtctctgaaccaaagaatcccatctttgagtcagttcctctgagtcactgttgatcttcttagatgccttggaattatcaagtaattgtcccacatcctggccaatctcactcagctgatccaatgtttgacgcttcatttccatgtcttccttcaaaatagccagacgtcgaacactgacacttagttccttttggtctttgaagttgcttgtctggactttatttaaagcctcttctttttcggttaaccaagctttcaacaagcactgttcttccaataattcctgccacaatatattgatttcttgtaacctattccagcgttcttcagtccaacggcatactgctgtccagcgctcaccaagtttctgtaactggtcttctaggatagctgtagcactctcaccactgttttcatcaacaatgaccaccatgtgagttagtgaatttactttcacctgttcagcctcaagatcactttgcaaacttttatgttcttctagcagcttttgtagagattttacatcatcatccagggggcaagtttccatcttctgaatgcgctcctctgtgagtgttaaccaggcggagagctgctgcagttgcttcttctgcagttccatcagcacatcgtgcagccgggactgtctgtccatactctccaccctaagagcctcccatctagcattcagcagggtcatctgttcctgaatctcaaattcttcttcgtctgacagagttccttgtgttatcagttggttgcctgcctgcaggacgctgcccacactgctctggtgtgcagtcagttccatcataaaagcttcatgggttgcaaactggtctttgacttcttcaacatcatcagaaatatcatcctgctcctggaaagtgtcctcagcagaaagcaaccaggtcagcacttcctccaacgcaatctgatagctgtccagatccatgtcaacctcagtgacagtgctgggagtttcagctcggggactctcatgctcctcctcaggcgctgtactctgtatattaattgcctcttcttcacattcttttttatatttccttgggagtgtctctacctcacggatggcgtctatggtgacttgctgaggtagcacctcaaacaaagatgttaaatacataattatggatttcttgtcaggaagctgaacggcaacatcttcaggatctaacagcttttcaattcccaaataagtttgagccttgctgaaggcatgttcaagtctctcaattggtgacattttgacaactttatcccagctgaagagatcaggtttatgtcggtggaggacagcattaaaggcgagtccatctgtccagctggtggtgaagttgaggacgttgacttggctgtagggcctggtggtctgacgcacccagctgagcaggatcttctcactgttcgtctgctgcaggtccgacatgacatccttcatgacatctttcacctgccagtgcaaaatgatgctccaaagtaaccccaaagtcagtttgtgatttccatccacaatgtcagttccccctatattcactaattccacattgttctgatgtaaaacctgcagcactctgttgacgttatttaaggcatgtacccttgtggaaccacgttcctttggcagtgatgttcctgtgaggccttctagaagatccaatagcttccttccatctttgaggtctgtgaacatatcattgatgggtggtttcccactctttgaaaatcgagcatttatccatttggtaaaggttttcttctgtacgtcattgtgttcatcagatctggacttaatgatatcactgaattcgttctgcccattgtcaggactggcttcatgttctccatacttggccatcttgccagagtttcaagataatccaaaaactttaccaagtcctctttctaaggctttcaacttcctacgatggttcagcttgacatcaataccttgtcagttgcagcaagagatccccagagtccggaaaaggagagccggcgactgcgcgggactacacaccaatggggcgcccccctcctcctgtcccctcagtctctccagggccgctgccagggagcttggcgatcgcgccacactctccggagccccacccttgggagcagcaaccacccagaggtcaagcacgttccccgccgggcggctggct

SEQ ID NO: 10737 - RNA, 11140 nt, Homo sapiens
  source 1..11140: mol_type = other RNA
ctcatctgcaaagaagtaagtgggcaacgtcaaataaagttaaacggcatacacagggctgtagcttaaaccatatgtgtgtatatataagatatttgattgaaatttatgaatttattaatgtggccaaatcacggaaacaaatacatggatctatttgggatctagttggttatatggctgataaacatatggctgataaattataaataaccaaaacattgtggtaaaagagtcaaagaaaaaatgaagtaattgtgcaaggttaatatgaacagcagaaggaatgtaaaaatgtaaagtggtcttctaattcttatgtaagctttgtcatagttattaaaaagacggtatcatattagaaagcccccacccactttcccaatgctgtatacattatacaaatccgtgacaaatgtattaccatttccaaatacctctctgttcattaatttacacttgcatagaaagggaagaagaaaacaataatatatggttattataaaaacaaaatatccatttctctttggatagtcagtgttttactctttcagtagaacacacagtcagcactcaacatcgtgggccaaggagccatggagcttctgatttaatggaacttggaattggcatttgctgaaaagggcaacactgtacgtcaggaaacattggttggccggatgaatacttcacattgcctgtggcctgctgggaacatttgggcagcaagatggaaacgtgctgtgaatctgctccatgacctccgtgagatccgtgctggtgtcgtgcggtggggccagcaggtcctctcccgctgcctggtggaactgtgggccggaggcatctggatcaagcgagtagctcagtgcagaatgctgaggagaagcccatggggaaacaccattgattcgggaatcagattcaggctgctccagcagctgtcggaggcggtggagctgagactccagctgtttattgtgatcttctaaaatctgcatcctagcctccagccgacctttgtgctgcctgaggagttttgcttctgctataagttctgaatcctcagacgtgtgatggggagatataatcgactctggcggtgaaccgacagggagcccccttcggaggtgctggtccttcagctgctcatactccacctgtagatttctttgttcttcctccaggtcagcaatgatcctctccagttctccacgttcttccctctctactgacttcaggatctgagctgggctctgcggctggctcactggggactctcctccgagtgtttggcaatactgctggatgagggcgtgctcgtcttccacacttcctgtggtggagctgctatcagtgagaaaagacccattagtcctttccatctgggccagtcgtgtggcatattgttctattcttgaatgggtgtcatcatgaaacagttgaggagattgtgaggggtcatagtgctctggccacatactgatgagtgtgataggagtctctaagttgtcaccttcaagaactgtctggacaggcaggtaaccaagtcgagggtgtttggcaaagtacttcttcgacctgaacttgttcttaagtacctttgtgaagtctcgtacatcttccccagatgttgtaggtatacaatattccaccattgggtaatgtaatttgtgaccttttgctgttcgacccgaaaagaaacaactctggcagacatcatagttaaaatgcttaaggcttctatacctgaacccgacaattggacattctttacagatgttgcatttggcctgatgttttgcagtctccgctgctgccactcgatgtaaaactgggagccaaaccatggactgtggttccaaatgcatccaatctataaactctttcacacttatttctggtttattgttattctgttggaagcagctgcgaacactaggctcaatattactgcctccaaaagctgctacttcacctagctgccgggggatctggatggcatcatgaagtaacaggcccagctgcctctggtcacacatttctgttggccctgcaacttccttaaagagatatctgtatttttcttccaagagacctttggagagagacattaatccaatcttcagactctgcactctaatttttccagttcgacccgtgtcatagacattgagcaaccaattgagacacatatcaacacagagtggaacgttgaccaggtccttatgcatttgctcaagtccatcataagttgttgtcagacagttgatgacatctggaacactgaggagctggtcattttggttcaacttgtgctgtttgaaaatttcatttgttgtactcaactctaagagatccaaacatagtgctttttgtagtcttcggattttgattgctgtacggtaggcagaaaaacgtacattattcaggtcagcaagggattgaaagagttcggtcattttaggatggtcccaacaggtggtctgtgtttgatggttgatgtaatagggcactttattatgtgaaatggatctttgccacggcagctggactgacgtagagagaaaatgctgagaggatggtccaaaatctctgtgggcttcctgaagctgtttaaggcgatcatccacagaaacctgtaaaagtttccatcgcatattaaggtcatctagctggcgagacatctttagagagggatgcaggtcaagtggagacagctgactggataaatcattcaccgttttaactttaaagttgattggtgcaatttcttctctaaatgccatgattttttcaatgtgatcctgcagcgagtcaatgagtaagtctcccacgggcttccagccattccgcacggactctgcctccttcatgtcagcgtccaggtcatccatagctccctgcaggtctctgagtttctccaatgccttgtccacttgcttttgccaattgctagttacagcatttagactttcccatttttctttgacttcagaagactgtttgcgcatggctttggcaatcttttgggctctctcctcaggagttaattctgtttttgattgtaggtttcttcttggctcttcaggggcctcaattggctgatcagccaagaaaactcgggcctggtcgacagcattcaggacagaatattctttctcctttaactcccgtctcagggccttacaatggtcatactggagctgtaaggctggaacatctcctccaataggcatttgtttcttaagctcttcatctttcatattcagccatttgatcagttcttctaaggacatcagcaacctgttccacttctcagcgctggcctccaaatgggccctgatgctagcagattttgcttttaagtcattccatctttggttcatatcatccagtcgatgttgaagcatagtagcctcttcagaatttcccaaagcttttaccatcttctgcctgtttccgtcaatgcttttaaatatgtcattgtgggcatcaatttctgcctggatgtcctgcatctgctgtttgagttccctggccaagatactatcctgaagagcattctcccgatgagaggcatccacaagcacattcactgtggtctctgcttcttggatccacttcaggaagttttccagatctctgcgagaggcctgcaccgtcctccactcagcctccaaggcgttctgtctgtcagcaatactttgtttgagattgatccatgatgtttttaagtactctgtggtttctttcacattccttgtgtcatcactcccatattcctccaggagtttctgcaggacgttatcgaacgccatgacgataccatctccaggacccagttcttgaagcagtatttggttatcagaaatttgtttggtgagtggatcccgtcgggcttgctgaagaatatagagtcgagcctcatattttctcatcagttcttcagtctcctccctatggtcatcccactgaagactgtcaataatcatgtcctcaagctgctgctgtcttagctcaacgccatgctgggtgccatcccactggttcttgaccctttccaatttttctgtaattgctgttctcatatctgaactggaagctttatttttcaaattctgtgccaatgtaaaaacataatccagctgaggatggcgctgttctaagtcagcctttgtaattttcattcgggaaacggtcttattgatctcttctacatccccaacagtgacaatgttggacttcagcatctggtcgattaataccagccagtcggctagttctgttatagttttatcaagatcagcaggaattgaaatttccgaagtacgatgagactgaacaggaatatctgacgcagatgatactagcaccaccttttggacattaggatgagcagcaatccttgtctgtgaaacagaactgggctcctggatgcattccttcagggtggtaggcacctctctgcaaatcttattccatgtcatatttacagtccttaagctttctgaaattttatccctttcaggtaaactcagacttttatctgaaagcatctccaattcagttctattcagccatttgagtttttcagcatgtacttccatttcttgagttaagtctcttaattcttgcaggttttctcccaattcggtggttgatctcttttgcatagcatgctcagcctttgttaaccaacagataatctcatctagctgatgcctgtacttcatcacctgcttactttctccttttagccttggctgcctatccttcacttctgcaacaattgcatcccagcgttggtttaaacctgccagtttttctttcaagaagcttccatctgcctgggagagtttctgcacaatcccatccccagttcggtttagtgctgcaaaactgggctggtggctgctgatgcccacctcaagttcctgctgatgtatcctggctttctctaagtccaggctgccacctggagcacaggtatcaaccagtaattcttcagcctctgttatccactgtgtgaggtcattaaggtcacaatggaactgtctccattcttccattgccctgtcaaaacaacctttccgatcactgtacattctattaattctgtcccattttgcattcagctgagtaagtgtatctctgatctgaatggcttcaggtccagaggcttcaaggatgacatctggctgtttttcatgaatgactgcaatctgctctccaagtttgtccagttggtctttgatattcttcagagagtcttcctgaaaagagaagtcttcgtaaatagcagtgttgagctctggaacattaagcgataattcaacatcatccatgcaaagtaaaattttgttaatttcaaccagataatctgtaggaagaagtgatgatctaattccagaagcaagttgacccattttcctctgttgaatagggattgccttaattttgttgtatctagtatgcaaaagtaataattgcaaacggatcttttcttttttattatcttccataggttgatgtaacatttcttctcctctttgtagaacttcctcaatctgggcactctcctcatccatcttttcatcttcatcactggattccaagtgtttttccacaaattttaacatattttctatgtcattttctaatttttccaagtcagagaaaggcacaccagtttcaaatgtttcagtggtgaccaaacattggtataatggttcctgagcaattagcaatttggcacttttgatatgttgagacaccttttcaaagttcctattcagctcagctaactttggttctacaagctccctgcttgagcttccacgggcattcatcaaaataagggcttgatcgcggacattttcaacctggaggttggcatcatccagctcagatactaaacgcttcacaatttcttcctgtttacttgttggtttcttttcaatttcatccaatagagcttcagcttgataaagccaggtacttatgtgagccacgttcccatcaaatatttctagctggttctgatggttcatcaaggtattgcaccaatcttcagtccaggtacgaactcggctccacccagcgttaaggacgcagagcctctcttctaaaataggctcactgccctcaatcaagttttgcagggcagcactactctctgtgatggtatttaaatcagcttttctcttttccagatccttcagaacatttttagcccaggaaatttctgtatccaagtcaccaagcagaccttctgaagtggacttctgtaccaattcagtttcagtagcagaaagccattcagagagagaagcagcctctttcttcattttccgggccaactgtgatgctctttccagatcctgttttccttctgtcacctgtgcgcccaggtcattgtaaagaaccttcagggaagtcagctgctcatccatcccttttgggttgtccgtttgctgtttctggacaatatgtcttcctgttttaatcacagtttccacttcaagtttgacttcactcaaagttttatacagtttcatacacttgtccaggtgcgtctgtatgacgtcagggtctacgtccttcacatccagaacgtgaagttctgctttcacgccatccagcacacgcttgcagtccagcatgcgctgctcgaagttagctggcttctggaaaagctggaactttgtggacacctctcggagtttcctctgtagcacatccatctgacttcctcctctggcagtcctactctctggggaggtcaggggctgagaacgcatatttcttctcaactcctctagggttagctcatgggctgagatctctgcttggattttctgagcttcctgtggaacttggaaagcatctatcctgtcagtcaggtatgtggtgagctgtttgtccagctcccccaagctctcttgcaagacttgaagcatctggtcagtttcccgcagcacctggagttgcttttccaaagaaatctgcttgctctctgccaggtgacttagatcttcatatcggctgttgaaagcctccagtttctcactgattatatcatccaggatccccccatcaatcagagtctggccaagctctcgaatctgggtgcgattatctgccgggtggcgcagaacagattccagagactccagggcttcgttgacagcatccgtcttctcaggcaggacctctgtgctcttcatccgctcttccaaagtgtttaaccaggtagtttcaagatccaaatagtgaagcagttcaatccaacaagaccagacctcctctagcgtgtggcactttcctcgaattctattacaaagaagttggtaattctccagcacaacattcagctcagacgtcaactcctggccaccagagggcaccttggcagctaataacttgatgttgtccttgagaatcttcactctcacctccttctgcaacacatcctcttttgccctcttcatctcttccacagcactctcaagctcttctggtgacttgtactcaaaatcccgctccaaatattcttcctcggcctgggtcatccattcctgcatctctgccaagtctttcttcaggttcgcagctttttcttgactttcagacaacctacttttttgagtagcgatctccttgctaagtttctccagttgagtttggtagtcacctagtcttgtctgcacccaagtttttattccagcaactggaccacttcgaagattagtctctatttccttcatgtttttcagagatgattcaattgtttctatttcattaacaaatgcagagcactggtctaactgcctctgtagacctgcgtcgtctccttgggcagcctgctgtttcattaagaagtctttcacgccatccatccacttctcaatgactgttgaatcggcctcaaaagctctgagtgtgagagcaatttcctcaagcaaatgtagatctttggaaaccaagacctttagcttgttccactttccttgcacatcatcaaattcttgcttatataatttttctacatcaggatgaacatttttctccagagcctttgtttcttctgcaagtttatgtaatgcaggtttctgattctcaaggatttcatcaagggtctttttttcttgcagggccttctccaccttggcaagatcattaaggacattcagagacacctgggccttattttctgaatcatttagcacatctttcagtgttttcaatgtttccagatatgcatgtccaggttggcccttcagttcattctctagatgttgttgacgatcctctacagcctcttgtacagcttggtagcggcccagaaagctatcgaagccccgctggacaaaatctggggcagaaggctgagacatcagggccgagcagcttgcacgagccatttcaattttggggtgaaggccaagaagatttgtcaattcccgctgacaggaatccttcaagcttggcaaggactgccgggaagattcagaaatggaagtgtgttttacccactcctcctttgtcttgatgaccttttcaagctcatcaagctgcttgaaataagcatttatatcttcctgtagctgaatctttctttctagatcttccaaatgttgagatacattcttccattctgatgaaaccttctccagaacattttttatttcttcagtaggaaggccttcttttcccatttgctccacaaggatttgtccagtttggtttaattcatctgctctggggattctttctctctgttctttttctaatgccttcaacttctttttcatttcggaagtgtcttgcatcttcatatactcttttatctctgtggtctgaatggcagttttccatttcaaaatccagttcaacagctctgcacttatagcatcaaactttttcttagcttcaatatccacatggatctgtctcttctttgggggaggaggaggaggcagttcctgcttagatttttttgtaattgcttgttctcttacacgaacagtctccaaaaggtccttctgaggaatctgagacatccccagctttgctacagcctgagtcacctggttggaggaatcttctagtctctgaaccaaagaatcccatctttgagtcagttcctctgagtcactgttgatcttcttagatgccttggaattatcaagtaattgtcccacatcctggccaatctcactcagctgatccaatgtttgacgcttcatttccatgtcttccttcaaaatagccagacgtcgaacactgacacttagttccttttggtctttgaagttgcttgtctggactttatttaaagcctcttctttttcggttaaccaagctttcaacaagcactgttcttccaataattcctgccacaatatattgatttcttgtaacctattccagcgttcttcagtccaacggcatactgctgtccagcgctcaccaagtttctgtaactggtcttctaggatagctgtagcactctcaccactgttttcatcaacaatgaccaccatgtgagttagtgaatttactttcacctgttcagcctcaagatcactttgcaaacttttatgttcttctagcagcttttgtagagattttacatcatcatccagggggcaagtttccatcttctgaatgcgctcctctgtgagtgttaaccaggcggagagctgctgcagttgcttcttctgcagttccatcagcacatcgtgcagccgggactgtctgtccatactctccaccctaagagcctcccatctagcattcagcagggtcatctgttcctgaatctcaaattcttcttcgtctgacagagttccttgtgttatcagttggttgcctgcctgcaggacgctgcccacactgctctggtgtgcagtcagttccatcataaaagcttcatgggttgcaaactggtctttgacttcttcaacatcatcagaaatatcatcctgctcctggaaagtgtcctcagcagaaagcaaccaggtcagcacttcctccaacgcaatctgatagctgtccagatccatgtcaacctcagtgacagtgctgggagtttcagctcggggactctcatgctcctcctcaggcgctgtactctgtatattaattgcctcttcttcacattcttttttatatttccttgggagtgtctctacctcacggatggcgtctatggtgacttgctgaggtagcacctcaaacaaagatgttaaatacataattatggatttcttgtcaggaagctgaacggcaacatcttcaggatctaacagcttttcaattcccaaataagtttgagccttgctgaaggcatgttcaagtctctcaattggtgacattttgacaactttatcccagctgaagagatcaggtttatgtcggtggaggacagcattaaaggcgagtccatctgtccagctggtggtgaagttgaggacgttgacttggctgtagggcctggtggtctgacgcacccagctgagcaggatcttctcactgttcgtctgctgcaggtccgacatgacatccttcatgacatctttcacctgccagtgcaaaatgatgctccaaagtaaccccaaagtcagtttgtgatttccatccacaatgtcagttccccctatattcactaattccacattgttctgatgtaaaacctgcagcactctgttgacgttatttaaggcatgtacccttgtggaaccacgttcctttggcagtgatgttcctgtgaggccttctagaagatccaatagcttccttccatctttgaggtctgtgaacatatcattgatgggtggtttcccactctttgaaaatcgagcatttatccatttggtaaaggttttcttctgtacgtcattgtgttcatcctgacgatggcaggggtaatggaaacccagatcttgagggccaagtctcatcccttaaagaactgctcagggccaggcgccgtggctcatgcctgtaatcccagcactttgggaggctgaggcgggcggatcacgaggtcaggagatccagaccatcctggctaacacggggaaaccccgtctctactaaaaatacaaaaaattagccgggcgtgatggcgggcgcc

SEQ ID NO: 10738 - RNA, 12103 nt, Homo sapiens
  source 1..12103: mol_type = other RNA
ctcatctgcaaagaagtaagtgggcaacgtcaaataaagttaaacggcatacacagggctgtagcttaaaccatatgtgtgtatatataagatatttgattgaaatttatgaatttattaatgtggccaaatcacggaaacaaatacatggatctatttgggatctagttggttatatggctgataaacatatggctgataaattataaataaccaaaacattgtggtaaaagagtcaaagaaaaaatgaagtaattgtgcaaggttaatatgaacagcagaaggaatgtaaaaatgtaaagtggtcttctaattcttatgtaagctttgtcatagttattaaaaagacggtatcatattagaaagcccccacccactttcccaatgctgtatacattatacaaatccgtgacaaatgtattaccatttccaaatacctctctgttcattaatttacacttgcatagaaagggaagaagaaaacaataatatatggttattataaaaacaaaatatccatttctctttggatagtcagtgttttactctttcagtagaacacacagtcagcactcaacatcgtgggccaaggagccatggagcttctgatttaatggaacttggaattggcatttgctgaaaagggcaacactgtacgtcaggaaacattggttggccggatgaatacttcacattgcctgtggcctgctgggaacatttgggcagcaagatggaaacgtgctgtgaatctgctccatgacctccgtgagatccgtgctggtgtcgtgcggtggggccagcaggtcctctcccgctgcctggtggaactgtgggccggaggcatctggatcaagcgagtagctcagtgcagaatgctgaggagaagcccatggggaaacaccattgattcgggaatcagattcaggctgctccagcagctgtcggaggcggtggagctgagactccagctgtttattgtgatcttctaaaatctgcatcctagcctccagccgacctttgtgctgcctgaggagttttgcttctgctataagttctgaatcctcagacgtgtgatggggagatataatcgactctggcggtgaaccgacagggagcccccttcggaggtgctggtccttcagctgctcatactccacctgtagatttctttgttcttcctccaggtcagcaatgatcctctccagttctccacgttcttccctctctactgacttcaggatctgagctgggctctgcggctggctcactggggactctcctccgagtgtttggcaatactgctggatgagggcgtgctcgtcttccacacttcctgtggtggagctgctatcagtgagaaaagacccattagtcctttccatctgggccagtcgtgtggcatattgttctattcttgaatgggtgtcatcatgaaacagttgaggagattgtgaggggtcatagtgctctggccacatactgatgagtgtgataggagtctctaagttgtcaccttcaagaactgtctggacaggcaggtaaccaagtcgagggtgtttggcaaagtacttcttcgacctgaacttgttcttaagtacctttgtgaagtctcgtacatcttccccagatgttgtaggtatacaatattccaccattgggtaatgtaatttgtgaccttttgctgttcgacccgaaaagaaacaactctggcagacatcatagttaaaatgcttaaggcttctatacctgaacccgacaattggacattctttacagatgttgcatttggcctgatgttttgcagtctccgctgctgccactcgatgtaaaactgggagccaaaccatggactgtggttccaaatgcatccaatctataaactctttcacacttatttctggtttattgttattctgttggaagcagctgcgaacactaggctcaatattactgcctccaaaagctgctacttcacctagctgccgggggatctggatggcatcatgaagtaacaggcccagctgcctctggtcacacatttctgttggccctgcaacttccttaaagagatatctgtatttttcttccaagagacctttggagagagacattaatccaatcttcagactctgcactctaatttttccagttcgacccgtgtcatagacattgagcaaccaattgagacacatatcaacacagagtggaacgttgaccaggtccttatgcatttgctcaagtccatcataagttgttgtcagacagttgatgacatctggaacactgaggagctggtcattttggttcaacttgtgctgtttgaaaatttcatttgttgtactcaactctaagagatccaaacatagtgctttttgtagtcttcggattttgattgctgtacggtaggcagaaaaacgtacattattcaggtcagcaagggattgaaagagttcggtcattttaggatggtcccaacaggtggtctgtgtttgatggttgatgtaatagggcactttattatgtgaaatggatctttgccacggcagctggactgacgtagagagaaaatgctgagaggatggtccaaaatctctgtgggcttcctgaagctgtttaaggcgatcatccacagaaacctgtaaaagtttccatcgcatattaaggtcatctagctggcgagacatctttagagagggatgcaggtcaagtggagacagctgactggataaatcattcaccgttttaactttaaagttgattggtgcaatttcttctctaaatgccatgattttttcaatgtgatcctgcagcgagtcaatgagtaagtctcccacgggcttccagccattccgcacggactctgcctccttcatgtcagcgtccaggtcatccatagctccctgcaggtctctgagtttctccaatgccttgtccacttgcttttgccaattgctagttacagcatttagactttcccatttttctttgacttcagaagactgtttgcgcatggctttggcaatcttttgggctctctcctcaggagttaattctgtttttgattgtaggtttcttcttggctcttcaggggcctcaattggctgatcagccaagaaaactcgggcctggtcgacagcattcaggacagaatattctttctcctttaactcccgtctcagggccttacaatggtcatactggagctgtaaggctggaacatctcctccaataggcatttgtttcttaagctcttcatctttcatattcagccatttgatcagttcttctaaggacatcagcaacctgttccacttctcagcgctggcctccaaatgggccctgatgctagcagattttgcttttaagtcattccatctttggttcatatcatccagtcgatgttgaagcatagtagcctcttcagaatttcccaaagcttttaccatcttctgcctgtttccgtcaatgcttttaaatatgtcattgtgggcatcaatttctgcctggatgtcctgcatctgctgtttgagttccctggccaagatactatcctgaagagcattctcccgatgagaggcatccacaagcacattcactgtggtctctgcttcttggatccacttcaggaagttttccagatctctgcgagaggcctgcaccgtcctccactcagcctccaaggcgttctgtctgtcagcaatactttgtttgagattgatccatgatgtttttaagtactctgtggtttctttcacattccttgtgtcatcactcccatattcctccaggagtttctgcaggacgttatcgaacgccatgacgataccatctccaggacccagttcttgaagcagtatttggttatcagaaatttgtttggtgagtggatcccgtcgggcttgctgaagaatatagagtcgagcctcatattttctcatcagttcttcagtctcctccctatggtcatcccactgaagactgtcaataatcatgtcctcaagctgctgctgtcttagctcaacgccatgctgggtgccatcccactggttcttgaccctttccaatttttctgtaattgctgttctcatatctgaactggaagctttatttttcaaattctgtgccaatgtaaaaacataatccagctgaggatggcgctgttctaagtcagcctttgtaattttcattcgggaaacggtcttattgatctcttctacatccccaacagtgacaatgttggacttcagcatctggtcgattaataccagccagtcggctagttctgttatagttttatcaagatcagcaggaattgaaatttccgaagtacgatgagactgaacaggaatatctgacgcagatgatactagcaccaccttttggacattaggatgagcagcaatccttgtctgtgaaacagaactgggctcctggatgcattccttcagggtggtaggcacctctctgcaaatcttattccatgtcatatttacagtccttaagctttctgaaattttatccctttcaggtaaactcagacttttatctgaaagcatctccaattcagttctattcagccatttgagtttttcagcatgtacttccatttcttgagttaagtctcttaattcttgcaggttttctcccaattcggtggttgatctcttttgcatagcatgctcagcctttgttaaccaacagataatctcatctagctgatgcctgtacttcatcacctgcttactttctccttttagccttggctgcctatccttcacttctgcaacaattgcatcccagcgttggtttaaacctgccagtttttctttcaagaagcttccatctgcctgggagagtttctgcacaatcccatccccagttcggtttagtgctgcaaaactgggctggtggctgctgatgcccacctcaagttcctgctgatgtatcctggctttctctaagtccaggctgccacctggagcacaggtatcaaccagtaattcttcagcctctgttatccactgtgtgaggtcattaaggtcacaatggaactgtctccattcttccattgccctgtcaaaacaacctttccgatcactgtacattctattaattctgtcccattttgcattcagctgagtaagtgtatctctgatctgaatggcttcaggtccagaggcttcaaggatgacatctggctgtttttcatgaatgactgcaatctgctctccaagtttgtccagttggtctttgatattcttcagagagtcttcctgaaaagagaagtcttcgtaaatagcagtgttgagctctggaacattaagcgataattcaacatcatccatgcaaagtaaaattttgttaatttcaaccagataatctgtaggaagaagtgatgatctaattccagaagcaagttgacccattttcctctgttgaatagggattgccttaattttgttgtatctagtatgcaaaagtaataattgcaaacggatcttttcttttttattatcttccataggttgatgtaacatttcttctcctctttgtagaacttcctcaatctgggcactctcctcatccatcttttcatcttcatcactggattccaagtgtttttccacaaattttaacatattttctatgtcattttctaatttttccaagtcagagaaaggcacaccagtttcaaatgtttcagtggtgaccaaacattggtataatggttcctgagcaattagcaatttggcacttttgatatgttgagacaccttttcaaagttcctattcagctcagctaactttggttctacaagctccctgcttgagcttccacgggcattcatcaaaataagggcttgatcgcggacattttcaacctggaggttggcatcatccagctcagatactaaacgcttcacaatttcttcctgtttacttgttggtttcttttcaatttcatccaatagagcttcagcttgataaagccaggtacttatgtgagccacgttcccatcaaatatttctagctggttctgatggttcatcaaggtattgcaccaatcttcagtccaggtacgaactcggctccacccagcgttaaggacgcagagcctctcttctaaaataggctcactgccctcaatcaagttttgcagggcagcactactctctgtgatggtatttaaatcagcttttctcttttccagatccttcagaacatttttagcccaggaaatttctgtatccaagtcaccaagcagaccttctgaagtggacttctgtaccaattcagtttcagtagcagaaagccattcagagagagaagcagcctctttcttcattttccgggccaactgtgatgctctttccagatcctgttttccttctgtcacctgtgcgcccaggtcattgtaaagaaccttcagggaagtcagctgctcatccatcccttttgggttgtccgtttgctgtttctggacaatatgtcttcctgttttaatcacagtttccacttcaagtttgacttcactcaaagttttatacagtttcatacacttgtccaggtgcgtctgtatgacgtcagggtctacgtccttcacatccagaacgtgaagttctgctttcacgccatccagcacacgcttgcagtccagcatgcgctgctcgaagttagctggcttctggaaaagctggaactttgtggacacctctcggagtttcctctgtagcacatccatctgacttcctcctctggcagtcctactctctggggaggtcaggggctgagaacgcatatttcttctcaactcctctagggttagctcatgggctgagatctctgcttggattttctgagcttcctgtggaacttggaaagcatctatcctgtcagtcaggtatgtggtgagctgtttgtccagctcccccaagctctcttgcaagacttgaagcatctggtcagtttcccgcagcacctggagttgcttttccaaagaaatctgcttgctctctgccaggtgacttagatcttcatatcggctgttgaaagcctccagtttctcactgattatatcatccaggatccccccatcaatcagagtctggccaagctctcgaatctgggtgcgattatctgccgggtggcgcagaacagattccagagactccagggcttcgttgacagcatccgtcttctcaggcaggacctctgtgctcttcatccgctcttccaaagtgtttaaccaggtagtttcaagatccaaatagtgaagcagttcaatccaacaagaccagacctcctctagcgtgtggcactttcctcgaattctattacaaagaagttggtaattctccagcacaacattcagctcagacgtcaactcctggccaccagagggcaccttggcagctaataacttgatgttgtccttgagaatcttcactctcacctccttctgcaacacatcctcttttgccctcttcatctcttccacagcactctcaagctcttctggtgacttgtactcaaaatcccgctccaaatattcttcctcggcctgggtcatccattcctgcatctctgccaagtctttcttcaggttcgcagctttttcttgactttcagacaacctacttttttgagtagcgatctccttgctaagtttctccagttgagtttggtagtcacctagtcttgtctgcacccaagtttttattccagcaactggaccacttcgaagattagtctctatttccttcatgtttttcagagatgattcaattgtttctatttcattaacaaatgcagagcactggtctaactgcctctgtagacctgcgtcgtctccttgggcagcctgctgtttcattaagaagtctttcacgccatccatccacttctcaatgactgttgaatcggcctcaaaagctctgagtgtgagagcaatttcctcaagcaaatgtagatctttggaaaccaagacctttagcttgttccactttccttgcacatcatcaaattcttgcttatataatttttctacatcaggatgaacatttttctccagagcctttgtttcttctgcaagtttatgtaatgcaggtttctgattctcaaggatttcatcaagggtctttttttcttgcagggccttctccaccttggcaagatcattaaggacattcagagacacctgggccttattttctgaatcatttagcacatctttcagtgttttcaatgtttccagatatgcatgtccaggttggcccttcagttcattctctagatgttgttgacgatcctctacagcctcttgtacagcttggtagcggcccagaaagctatcgaagccccgctggacaaaatctggggcagaaggctgagacatcagggccgagcagcttgcacgagccatttcaattttggggtgaaggccaagaagatttgtcaattcccgctgacaggaatccttcaagcttggcaaggactgccgggaagattcagaaatggaagtgtgttttacccactcctcctttgtcttgatgaccttttcaagctcatcaagctgcttgaaataagcatttatatcttcctgtagctgaatctttctttctagatcttccaaatgttgagatacattcttccattctgatgaaaccttctccagaacattttttatttcttcagtaggaaggccttcttttcccatttgctccacaaggatttgtccagtttggtttaattcatctgctctggggattctttctctctgttctttttctaatgccttcaacttctttttcatttcggaagtgtcttgcatcttcatatactcttttatctctgtggtctgaatggcagttttccatttcaaaatccagttcaacagctctgcacttatagcatcaaactttttcttagcttcaatatccacatggatctgtctcttctttgggggaggaggaggaggcagttcctgcttagatttttttgtaattgcttgttctcttacacgaacagtctccaaaaggtccttctgaggaatctgagacatccccagctttgctacagcctgagtcacctggttggaggaatcttctagtctctgaaccaaagaatcccatctttgagtcagttcctctgagtcactgttgatcttcttagatgccttggaattatcaagtaattgtcccacatcctggccaatctcactcagctgatccaatgtttgacgcttcatttccatgtcttccttcaaaatagccagacgtcgaacactgacacttagttccttttggtctttgaagttgcttgtctggactttatttaaagcctcttctttttcggttaaccaagctttcaacaagcactgttcttccaataattcctgccacaatatattgatttcttgtaacctattccagcgttcttcagtccaacggcatactgctgtccagcgctcaccaagtttctgtaactggtcttctaggatagctgtagcactctcaccactgttttcatcaacaatgaccaccatgtgagttagtgaatttactttcacctgttcagcctcaagatcactttgcaaacttttatgttcttctagcagcttttgtagagattttacatcatcatccagggggcaagtttccatcttctgaatgcgctcctctgtgagtgttaaccaggcggagagctgctgcagttgcttcttctgcagttccatcagcacatcgtgcagccgggactgtctgtccatactctccaccctaagagcctcccatctagcattcagcagggtcatctgttcctgaatctcaaattcttcttcgtctgacagagttccttgtgttatcagttggttgcctgcctgcaggacgctgcccacactgctctggtgtgcagtcagttccatcataaaagcttcatgggttgcaaactggtctttgacttcttcaacatcatcagaaatatcatcctgctcctggaaagtgtcctcagcagaaagcaaccaggtcagcacttcctccaacgcaatctgatagctgtccagatccatgtcaacctcagtgacagtgctgggagtttcagctcggggactctcatgctcctcctcaggcgctgtactctgtatattaattgcctcttcttcacattcttttttatatttccttgggagtgtctctacctcacggatggcgtctatggtgacttgctgaggtagcacctcaaacaaagatgttaaatacataattatggatttcttgtcaggaagctgaacggcaacatcttcaggatctaacagcttttcaattcccaaataagtttgagccttgctgaaggcatgttcaagtctctcaattggtgacattttgacaactttatcccagctgaagagatcaggtttatgtcggtggaggacagcattaaaggcgagtccatctgtccagctggtggtgaagttgaggacgttgacttggctgtagggcctggtggtctgacgcacccagctgagcaggatcttctcactgttcgtctgctgcaggtccgacatgacatccttcatgacatctttcacctgccagtgcaaaatgatgctccaaagtaaccccaaagtcagtttgtgatttccatccacaatgtcagttccccctatattcactaattccacattgttctgatgtaaaacctgcagcactctgttgacgttatttaaggcatgtacccttgtggaaccacgttcctttggcagtgatgttcctgtgaggccttctagaagatccaatagcttccttccatctttgaggtctgtgaacatatcattgatgggtggtttcccactctttgaaaatcgagcatttatccatttggtaaaggttttcttctgtacgtcattgtgttcatctgcctgtgactgtctgccgtctccgtttgtggattcagatctcacttccatttctcgtcggctcagcgtgtcctccaaatgtagttaagactcccaaaccaacagtgcatgatttctgaagtcacaaagggatgtgtacccctcggctggagaatgtgctttgatggagtcaaattgaaaaacagggccaaacagtatgggaaccgtggatagatgagttcctccccaactgcccggaccagaatggtcacattcctgcctctgtgaatagcccaatcctggtctgctctgtctgagcctctgccaggtgtggagcctgtcgccttaaaatctgaagacgtgtgacaacacttatctgcctaggaacagcaaggtatgcatttctacaaacaccactgttgaaactgcttggtatacagagaagccaagcacttcctctcttctcaggttttccttagattcaagccaaatagaaatctgagtgaggaaaaatgttaaggaatttagctttagaaaaatttgtttttatgtttctaactcttgcaagagagcttgttctcatcaattttataacctatttttcaacctacatactccagactaattcctaatgcttttagggatccatccattaatgcactaaataatacatgccctcaaactaagaggtaaaccatgccccttcaatcaggataagaaatactactgagtgaaatgcagactgcatctttctgccaattttaatccacagccctctgctcacttcactcccaatcaccggcctcaatcaggctttctgtgggccaagttctgccagcttagagcctgcacacagctctgccttcagccagtgccctccaccaccttgaactatggacttgaatagattcctcaagaaggccttccctgaccactcaaactatcactcattccaggtccctatgaagtccccgagtgatttgccatgacagcactgcagaatgtctaccctctaagcagttaaacaactatttgtatgctctgcaatttgatgtctggttctcgtactagtctacacactcaagaggccagatgccatcatagagctcatcagttttgtcaactacacccagtgcagtgcctgccatatggggcattcacccaagactactttccatttaaaattgttgtctcttttgaaacactctgtg

SEQ ID NO: 10739 - RNA, 11021 nt, Homo sapiens
  source 1..11021: mol_type = other RNA
ctcatctgcaaagaagtaagtgggcaacgtcaaataaagttaaacggcatacacagggctgtagcttaaaccatatgtgtgtatatataagatatttgattgaaatttatgaatttattaatgtggccaaatcacggaaacaaatacatggatctatttgggatctagttggttatatggctgataaacatatggctgataaattataaataaccaaaacattgtggtaaaagagtcaaagaaaaaatgaagtaattgtgcaaggttaatatgaacagcagaaggaatgtaaaaatgtaaagtggtcttctaattcttatgtaagctttgtcatagttattaaaaagacggtatcatattagaaagcccccacccactttcccaatgctgtatacattatacaaatccgtgacaaatgtattaccatttccaaatacctctctgttcattaatttacacttgcatagaaagggaagaagaaaacaataatatatggttattataaaaacaaaatatccatttctctttggatagtcagtgttttactctttcagtagaacacacagtcagcactcaacatcgtgggccaaggagccatggagcttctgatttaatggaacttggaattggcatttgctgaaaagggcaacactgtacgtcaggaaacattggttggccggatgaatacttcacattgcctgtggcctgctgggaacatttgggcagcaagatggaaacgtgctgtgaatctgctccatgacctccgtgagatccgtgctggtgtcgtgcggtggggccagcaggtcctctcccgctgcctggtggaactgtgggccggaggcatctggatcaagcgagtagctcagtgcagaatgctgaggagaagcccatggggaaacaccattgattcgggaatcagattcaggctgctccagcagctgtcggaggcggtggagctgagactccagctgtttattgtgatcttctaaaatctgcatcctagcctccagccgacctttgtgctgcctgaggagttttgcttctgctataagttctgaatcctcagacgtgtgatggggagatataatcgactctggcggtgaaccgacagggagcccccttcggaggtgctggtccttcagctgctcatactccacctgtagatttctttgttcttcctccaggtcagcaatgatcctctccagttctccacgttcttccctctctactgacttcaggatctgagctgggctctgcggctggctcactggggactctcctccgagtgtttggcaatactgctggatgagggcgtgctcgtcttccacacttcctgtggtggagctgctatcagtgagaaaagacccattagtcctttccatctgggccagtcgtgtggcatattgttctattcttgaatgggtgtcatcatgaaacagttgaggagattgtgaggggtcatagtgctctggccacatactgatgagtgtgataggagtctctaagttgtcaccttcaagaactgtctggacaggcaggtaaccaagtcgagggtgtttggcaaagtacttcttcgacctgaacttgttcttaagtacctttgtgaagtctcgtacatcttccccagatgttgtaggtatacaatattccaccattgggtaatgtaatttgtgaccttttgctgttcgacccgaaaagaaacaactctggcagacatcatagttaaaatgcttaaggcttctatacctgaacccgacaattggacattctttacagatgttgcatttggcctgatgttttgcagtctccgctgctgccactcgatgtaaaactgggagccaaaccatggactgtggttccaaatgcatccaatctataaactctttcacacttatttctggtttattgttattctgttggaagcagctgcgaacactaggctcaatattactgcctccaaaagctgctacttcacctagctgccgggggatctggatggcatcatgaagtaacaggcccagctgcctctggtcacacatttctgttggccctgcaacttccttaaagagatatctgtatttttcttccaagagacctttggagagagacattaatccaatcttcagactctgcactctaatttttccagttcgacccgtgtcatagacattgagcaaccaattgagacacatatcaacacagagtggaacgttgaccaggtccttatgcatttgctcaagtccatcataagttgttgtcagacagttgatgacatctggaacactgaggagctggtcattttggttcaacttgtgctgtttgaaaatttcatttgttgtactcaactctaagagatccaaacatagtgctttttgtagtcttcggattttgattgctgtacggtaggcagaaaaacgtacattattcaggtcagcaagggattgaaagagttcggtcattttaggatggtcccaacaggtggtctgtgtttgatggttgatgtaatagggcactttattatgtgaaatggatctttgccacggcagctggactgacgtagagagaaaatgctgagaggatggtccaaaatctctgtgggcttcctgaagctgtttaaggcgatcatccacagaaacctgtaaaagtttccatcgcatattaaggtcatctagctggcgagacatctttagagagggatgcaggtcaagtggagacagctgactggataaatcattcaccgttttaactttaaagttgattggtgcaatttcttctctaaatgccatgattttttcaatgtgatcctgcagcgagtcaatgagtaagtctcccacgggcttccagccattccgcacggactctgcctccttcatgtcagcgtccaggtcatccatagctccctgcaggtctctgagtttctccaatgccttgtccacttgcttttgccaattgctagttacagcatttagactttcccatttttctttgacttcagaagactgtttgcgcatggctttggcaatcttttgggctctctcctcaggagttaattctgtttttgattgtaggtttcttcttggctcttcaggggcctcaattggctgatcagccaagaaaactcgggcctggtcgacagcattcaggacagaatattctttctcctttaactcccgtctcagggccttacaatggtcatactggagctgtaaggctggaacatctcctccaataggcatttgtttcttaagctcttcatctttcatattcagccatttgatcagttcttctaaggacatcagcaacctgttccacttctcagcgctggcctccaaatgggccctgatgctagcagattttgcttttaagtcattccatctttggttcatatcatccagtcgatgttgaagcatagtagcctcttcagaatttcccaaagcttttaccatcttctgcctgtttccgtcaatgcttttaaatatgtcattgtgggcatcaatttctgcctggatgtcctgcatctgctgtttgagttccctggccaagatactatcctgaagagcattctcccgatgagaggcatccacaagcacattcactgtggtctctgcttcttggatccacttcaggaagttttccagatctctgcgagaggcctgcaccgtcctccactcagcctccaaggcgttctgtctgtcagcaatactttgtttgagattgatccatgatgtttttaagtactctgtggtttctttcacattccttgtgtcatcactcccatattcctccaggagtttctgcaggacgttatcgaacgccatgacgataccatctccaggacccagttcttgaagcagtatttggttatcagaaatttgtttggtgagtggatcccgtcgggcttgctgaagaatatagagtcgagcctcatattttctcatcagttcttcagtctcctccctatggtcatcccactgaagactgtcaataatcatgtcctcaagctgctgctgtcttagctcaacgccatgctgggtgccatcccactggttcttgaccctttccaatttttctgtaattgctgttctcatatctgaactggaagctttatttttcaaattctgtgccaatgtaaaaacataatccagctgaggatggcgctgttctaagtcagcctttgtaattttcattcgggaaacggtcttattgatctcttctacatccccaacagtgacaatgttggacttcagcatctggtcgattaataccagccagtcggctagttctgttatagttttatcaagatcagcaggaattgaaatttccgaagtacgatgagactgaacaggaatatctgacgcagatgatactagcaccaccttttggacattaggatgagcagcaatccttgtctgtgaaacagaactgggctcctggatgcattccttcagggtggtaggcacctctctgcaaatcttattccatgtcatatttacagtccttaagctttctgaaattttatccctttcaggtaaactcagacttttatctgaaagcatctccaattcagttctattcagccatttgagtttttcagcatgtacttccatttcttgagttaagtctcttaattcttgcaggttttctcccaattcggtggttgatctcttttgcatagcatgctcagcctttgttaaccaacagataatctcatctagctgatgcctgtacttcatcacctgcttactttctccttttagccttggctgcctatccttcacttctgcaacaattgcatcccagcgttggtttaaacctgccagtttttctttcaagaagcttccatctgcctgggagagtttctgcacaatcccatccccagttcggtttagtgctgcaaaactgggctggtggctgctgatgcccacctcaagttcctgctgatgtatcctggctttctctaagtccaggctgccacctggagcacaggtatcaaccagtaattcttcagcctctgttatccactgtgtgaggtcattaaggtcacaatggaactgtctccattcttccattgccctgtcaaaacaacctttccgatcactgtacattctattaattctgtcccattttgcattcagctgagtaagtgtatctctgatctgaatggcttcaggtccagaggcttcaaggatgacatctggctgtttttcatgaatgactgcaatctgctctccaagtttgtccagttggtctttgatattcttcagagagtcttcctgaaaagagaagtcttcgtaaatagcagtgttgagctctggaacattaagcgataattcaacatcatccatgcaaagtaaaattttgttaatttcaaccagataatctgtaggaagaagtgatgatctaattccagaagcaagttgacccattttcctctgttgaatagggattgccttaattttgttgtatctagtatgcaaaagtaataattgcaaacggatcttttcttttttattatcttccataggttgatgtaacatttcttctcctctttgtagaacttcctcaatctgggcactctcctcatccatcttttcatcttcatcactggattccaagtgtttttccacaaattttaacatattttctatgtcattttctaatttttccaagtcagagaaaggcacaccagtttcaaatgtttcagtggtgaccaaacattggtataatggttcctgagcaattagcaatttggcacttttgatatgttgagacaccttttcaaagttcctattcagctcagctaactttggttctacaagctccctgcttgagcttccacgggcattcatcaaaataagggcttgatcgcggacattttcaacctggaggttggcatcatccagctcagatactaaacgcttcacaatttcttcctgtttacttgttggtttcttttcaatttcatccaatagagcttcagcttgataaagccaggtacttatgtgagccacgttcccatcaaatatttctagctggttctgatggttcatcaaggtattgcaccaatcttcagtccaggtacgaactcggctccacccagcgttaaggacgcagagcctctcttctaaaataggctcactgccctcaatcaagttttgcagggcagcactactctctgtgatggtatttaaatcagcttttctcttttccagatccttcagaacatttttagcccaggaaatttctgtatccaagtcaccaagcagaccttctgaagtggacttctgtaccaattcagtttcagtagcagaaagccattcagagagagaagcagcctctttcttcattttccgggccaactgtgatgctctttccagatcctgttttccttctgtcacctgtgcgcccaggtcattgtaaagaaccttcagggaagtcagctgctcatccatcccttttgggttgtccgtttgctgtttctggacaatatgtcttcctgttttaatcacagtttccacttcaagtttgacttcactcaaagttttatacagtttcatacacttgtccaggtgcgtctgtatgacgtcagggtctacgtccttcacatccagaacgtgaagttctgctttcacgccatccagcacacgcttgcagtccagcatgcgctgctcgaagttagctggcttctggaaaagctggaactttgtggacacctctcggagtttcctctgtagcacatccatctgacttcctcctctggcagtcctactctctggggaggtcaggggctgagaacgcatatttcttctcaactcctctagggttagctcatgggctgagatctctgcttggattttctgagcttcctgtggaacttggaaagcatctatcctgtcagtcaggtatgtggtgagctgtttgtccagctcccccaagctctcttgcaagacttgaagcatctggtcagtttcccgcagcacctggagttgcttttccaaagaaatctgcttgctctctgccaggtgacttagatcttcatatcggctgttgaaagcctccagtttctcactgattatatcatccaggatccccccatcaatcagagtctggccaagctctcgaatctgggtgcgattatctgccgggtggcgcagaacagattccagagactccagggcttcgttgacagcatccgtcttctcaggcaggacctctgtgctcttcatccgctcttccaaagtgtttaaccaggtagtttcaagatccaaatagtgaagcagttcaatccaacaagaccagacctcctctagcgtgtggcactttcctcgaattctattacaaagaagttggtaattctccagcacaacattcagctcagacgtcaactcctggccaccagagggcaccttggcagctaataacttgatgttgtccttgagaatcttcactctcacctccttctgcaacacatcctcttttgccctcttcatctcttccacagcactctcaagctcttctggtgacttgtactcaaaatcccgctccaaatattcttcctcggcctgggtcatccattcctgcatctctgccaagtctttcttcaggttcgcagctttttcttgactttcagacaacctacttttttgagtagcgatctccttgctaagtttctccagttgagtttggtagtcacctagtcttgtctgcacccaagtttttattccagcaactggaccacttcgaagattagtctctatttccttcatgtttttcagagatgattcaattgtttctatttcattaacaaatgcagagcactggtctaactgcctctgtagacctgcgtcgtctccttgggcagcctgctgtttcattaagaagtctttcacgccatccatccacttctcaatgactgttgaatcggcctcaaaagctctgagtgtgagagcaatttcctcaagcaaatgtagatctttggaaaccaagacctttagcttgttccactttccttgcacatcatcaaattcttgcttatataatttttctacatcaggatgaacatttttctccagagcctttgtttcttctgcaagtttatgtaatgcaggtttctgattctcaaggatttcatcaagggtctttttttcttgcagggccttctccaccttggcaagatcattaaggacattcagagacacctgggccttattttctgaatcatttagcacatctttcagtgttttcaatgtttccagatatgcatgtccaggttggcccttcagttcattctctagatgttgttgacgatcctctacagcctcttgtacagcttggtagcggcccagaaagctatcgaagccccgctggacaaaatctggggcagaaggctgagacatcagggccgagcagcttgcacgagccatttcaattttggggtgaaggccaagaagatttgtcaattcccgctgacaggaatccttcaagcttggcaaggactgccgggaagattcagaaatggaagtgtgttttacccactcctcctttgtcttgatgaccttttcaagctcatcaagctgcttgaaataagcatttatatcttcctgtagctgaatctttctttctagatcttccaaatgttgagatacattcttccattctgatgaaaccttctccagaacattttttatttcttcagtaggaaggccttcttttcccatttgctccacaaggatttgtccagtttggtttaattcatctgctctggggattctttctctctgttctttttctaatgccttcaacttctttttcatttcggaagtgtcttgcatcttcatatactcttttatctctgtggtctgaatggcagttttccatttcaaaatccagttcaacagctctgcacttatagcatcaaactttttcttagcttcaatatccacatggatctgtctcttctttgggggaggaggaggaggcagttcctgcttagatttttttgtaattgcttgttctcttacacgaacagtctccaaaaggtccttctgaggaatctgagacatccccagctttgctacagcctgagtcacctggttggaggaatcttctagtctctgaaccaaagaatcccatctttgagtcagttcctctgagtcactgttgatcttcttagatgccttggaattatcaagtaattgtcccacatcctggccaatctcactcagctgatccaatgtttgacgcttcatttccatgtcttccttcaaaatagccagacgtcgaacactgacacttagttccttttggtctttgaagttgcttgtctggactttatttaaagcctcttctttttcggttaaccaagctttcaacaagcactgttcttccaataattcctgccacaatatattgatttcttgtaacctattccagcgttcttcagtccaacggcatactgctgtccagcgctcaccaagtttctgtaactggtcttctaggatagctgtagcactctcaccactgttttcatcaacaatgaccaccatgtgagttagtgaatttactttcacctgttcagcctcaagatcactttgcaaacttttatgttcttctagcagcttttgtagagattttacatcatcatccagggggcaagtttccatcttctgaatgcgctcctctgtgagtgttaaccaggcggagagctgctgcagttgcttcttctgcagttccatcagcacatcgtgcagccgggactgtctgtccatactctccaccctaagagcctcccatctagcattcagcagggtcatctgttcctgaatctcaaattcttcttcgtctgacagagttccttgtgttatcagttggttgcctgcctgcaggacgctgcccacactgctctggtgtgcagtcagttccatcataaaagcttcatgggttgcaaactggtctttgacttcttcaacatcatcagaaatatcatcctgctcctggaaagtgtcctcagcagaaagcaaccaggtcagcacttcctccaacgcaatctgatagctgtccagatccatgtcaacctcagtgacagtgctgggagtttcagctcggggactctcatgctcctcctcaggcgctgtactctgtatattaattgcctcttcttcacattcttttttatatttccttgggagtgtctctacctcacggatggcgtctatggtgacttgctgaggtagcacctcaaacaaagatgttaaatacataattatggatttcttgtcaggaagctgaacggcaacatcttcaggatctaacagcttttcaattcccaaataagtttgagccttgctgaaggcatgttcaagtctctcaattggtgacattttgacaactttatcccagctgaagagatcaggtttatgtcggtggaggacagcattaaaggcgagtccatctgtccagctggtggtgaagttgaggacgttgacttggctgtagggcctggtggtctgacgcacccagctgagcaggatcttctcactgttcgtctgctgcaggtccgacatgacatccttcatgacatctttcacctgccagtgcaaaatgatgctccaaagtaaccccaaagtcagtttgtgatttccatccacaatgtcagttccccctatattcactaattccacattgttctgatgtaaaacctgcagcactctgttgacgttatttaaggcatgtacccttgtggaaccacgttcctttggcagtgatgttcctgtgaggccttctagaagatccaatagcttccttccatctttgaggtctgtgaacatatcattgatgggtggtttcccactctttgaaaatcgagcatttatccatttggtaaaggttttcttctgtacgtcattgtgttcatctggtaatcgcttgcaagcctggagagctacatgccctggcaaatccaatctgcactttttccaatgaaacgtggtggctgccaggccgctcatcacctacatctgctt

SEQ ID NO: 10740 - RNA, 11300 nt, Homo sapiens
  source 1..11300: mol_type = other RNA
ctcatctgcaaagaagtaagtgggcaacgtcaaataaagttaaacggcatacacagggctgtagcttaaaccatatgtgtgtatatataagatatttgattgaaatttatgaatttattaatgtggccaaatcacggaaacaaatacatggatctatttgggatctagttggttatatggctgataaacatatggctgataaattataaataaccaaaacattgtggtaaaagagtcaaagaaaaaatgaagtaattgtgcaaggttaatatgaacagcagaaggaatgtaaaaatgtaaagtggtcttctaattcttatgtaagctttgtcatagttattaaaaagacggtatcatattagaaagcccccacccactttcccaatgctgtatacattatacaaatccgtgacaaatgtattaccatttccaaatacctctctgttcattaatttacacttgcatagaaagggaagaagaaaacaataatatatggttattataaaaacaaaatatccatttctctttggatagtcagtgttttactctttcagtagaacacacagtcagcactcaacatcgtgggccaaggagccatggagcttctgatttaatggaacttggaattggcatttgctgaaaagggcaacactgtacgtcaggaaacattggttggccggatgaatacttcacattgcctgtggcctgctgggaacatttgggcagcaagatggaaacgtgctgtgaatctgctccatgacctccgtgagatccgtgctggtgtcgtgcggtggggccagcaggtcctctcccgctgcctggtggaactgtgggccggaggcatctggatcaagcgagtagctcagtgcagaatgctgaggagaagcccatggggaaacaccattgattcgggaatcagattcaggctgctccagcagctgtcggaggcggtggagctgagactccagctgtttattgtgatcttctaaaatctgcatcctagcctccagccgacctttgtgctgcctgaggagttttgcttctgctataagttctgaatcctcagacgtgtgatggggagatataatcgactctggcggtgaaccgacagggagcccccttcggaggtgctggtccttcagctgctcatactccacctgtagatttctttgttcttcctccaggtcagcaatgatcctctccagttctccacgttcttccctctctactgacttcaggatctgagctgggctctgcggctggctcactggggactctcctccgagtgtttggcaatactgctggatgagggcgtgctcgtcttccacacttcctgtggtggagctgctatcagtgagaaaagacccattagtcctttccatctgggccagtcgtgtggcatattgttctattcttgaatgggtgtcatcatgaaacagttgaggagattgtgaggggtcatagtgctctggccacatactgatgagtgtgataggagtctctaagttgtcaccttcaagaactgtctggacaggcaggtaaccaagtcgagggtgtttggcaaagtacttcttcgacctgaacttgttcttaagtacctttgtgaagtctcgtacatcttccccagatgttgtaggtatacaatattccaccattgggtaatgtaatttgtgaccttttgctgttcgacccgaaaagaaacaactctggcagacatcatagttaaaatgcttaaggcttctatacctgaacccgacaattggacattctttacagatgttgcatttggcctgatgttttgcagtctccgctgctgccactcgatgtaaaactgggagccaaaccatggactgtggttccaaatgcatccaatctataaactctttcacacttatttctggtttattgttattctgttggaagcagctgcgaacactaggctcaatattactgcctccaaaagctgctacttcacctagctgccgggggatctggatggcatcatgaagtaacaggcccagctgcctctggtcacacatttctgttggccctgcaacttccttaaagagatatctgtatttttcttccaagagacctttggagagagacattaatccaatcttcagactctgcactctaatttttccagttcgacccgtgtcatagacattgagcaaccaattgagacacatatcaacacagagtggaacgttgaccaggtccttatgcatttgctcaagtccatcataagttgttgtcagacagttgatgacatctggaacactgaggagctggtcattttggttcaacttgtgctgtttgaaaatttcatttgttgtactcaactctaagagatccaaacatagtgctttttgtagtcttcggattttgattgctgtacggtaggcagaaaaacgtacattattcaggtcagcaagggattgaaagagttcggtcattttaggatggtcccaacaggtggtctgtgtttgatggttgatgtaatagggcactttattatgtgaaatggatctttgccacggcagctggactgacgtagagagaaaatgctgagaggatggtccaaaatctctgtgggcttcctgaagctgtttaaggcgatcatccacagaaacctgtaaaagtttccatcgcatattaaggtcatctagctggcgagacatctttagagagggatgcaggtcaagtggagacagctgactggataaatcattcaccgttttaactttaaagttgattggtgcaatttcttctctaaatgccatgattttttcaatgtgatcctgcagcgagtcaatgagtaagtctcccacgggcttccagccattccgcacggactctgcctccttcatgtcagcgtccaggtcatccatagctccctgcaggtctctgagtttctccaatgccttgtccacttgcttttgccaattgctagttacagcatttagactttcccatttttctttgacttcagaagactgtttgcgcatggctttggcaatcttttgggctctctcctcaggagttaattctgtttttgattgtaggtttcttcttggctcttcaggggcctcaattggctgatcagccaagaaaactcgggcctggtcgacagcattcaggacagaatattctttctcctttaactcccgtctcagggccttacaatggtcatactggagctgtaaggctggaacatctcctccaataggcatttgtttcttaagctcttcatctttcatattcagccatttgatcagttcttctaaggacatcagcaacctgttccacttctcagcgctggcctccaaatgggccctgatgctagcagattttgcttttaagtcattccatctttggttcatatcatccagtcgatgttgaagcatagtagcctcttcagaatttcccaaagcttttaccatcttctgcctgtttccgtcaatgcttttaaatatgtcattgtgggcatcaatttctgcctggatgtcctgcatctgctgtttgagttccctggccaagatactatcctgaagagcattctcccgatgagaggcatccacaagcacattcactgtggtctctgcttcttggatccacttcaggaagttttccagatctctgcgagaggcctgcaccgtcctccactcagcctccaaggcgttctgtctgtcagcaatactttgtttgagattgatccatgatgtttttaagtactctgtggtttctttcacattccttgtgtcatcactcccatattcctccaggagtttctgcaggacgttatcgaacgccatgacgataccatctccaggacccagttcttgaagcagtatttggttatcagaaatttgtttggtgagtggatcccgtcgggcttgctgaagaatatagagtcgagcctcatattttctcatcagttcttcagtctcctccctatggtcatcccactgaagactgtcaataatcatgtcctcaagctgctgctgtcttagctcaacgccatgctgggtgccatcccactggttcttgaccctttccaatttttctgtaattgctgttctcatatctgaactggaagctttatttttcaaattctgtgccaatgtaaaaacataatccagctgaggatggcgctgttctaagtcagcctttgtaattttcattcgggaaacggtcttattgatctcttctacatccccaacagtgacaatgttggacttcagcatctggtcgattaataccagccagtcggctagttctgttatagttttatcaagatcagcaggaattgaaatttccgaagtacgatgagactgaacaggaatatctgacgcagatgatactagcaccaccttttggacattaggatgagcagcaatccttgtctgtgaaacagaactgggctcctggatgcattccttcagggtggtaggcacctctctgcaaatcttattccatgtcatatttacagtccttaagctttctgaaattttatccctttcaggtaaactcagacttttatctgaaagcatctccaattcagttctattcagccatttgagtttttcagcatgtacttccatttcttgagttaagtctcttaattcttgcaggttttctcccaattcggtggttgatctcttttgcatagcatgctcagcctttgttaaccaacagataatctcatctagctgatgcctgtacttcatcacctgcttactttctccttttagccttggctgcctatccttcacttctgcaacaattgcatcccagcgttggtttaaacctgccagtttttctttcaagaagcttccatctgcctgggagagtttctgcacaatcccatccccagttcggtttagtgctgcaaaactgggctggtggctgctgatgcccacctcaagttcctgctgatgtatcctggctttctctaagtccaggctgccacctggagcacaggtatcaaccagtaattcttcagcctctgttatccactgtgtgaggtcattaaggtcacaatggaactgtctccattcttccattgccctgtcaaaacaacctttccgatcactgtacattctattaattctgtcccattttgcattcagctgagtaagtgtatctctgatctgaatggcttcaggtccagaggcttcaaggatgacatctggctgtttttcatgaatgactgcaatctgctctccaagtttgtccagttggtctttgatattcttcagagagtcttcctgaaaagagaagtcttcgtaaatagcagtgttgagctctggaacattaagcgataattcaacatcatccatgcaaagtaaaattttgttaatttcaaccagataatctgtaggaagaagtgatgatctaattccagaagcaagttgacccattttcctctgttgaatagggattgccttaattttgttgtatctagtatgcaaaagtaataattgcaaacggatcttttcttttttattatcttccataggttgatgtaacatttcttctcctctttgtagaacttcctcaatctgggcactctcctcatccatcttttcatcttcatcactggattccaagtgtttttccacaaattttaacatattttctatgtcattttctaatttttccaagtcagagaaaggcacaccagtttcaaatgtttcagtggtgaccaaacattggtataatggttcctgagcaattagcaatttggcacttttgatatgttgagacaccttttcaaagttcctattcagctcagctaactttggttctacaagctccctgcttgagcttccacgggcattcatcaaaataagggcttgatcgcggacattttcaacctggaggttggcatcatccagctcagatactaaacgcttcacaatttcttcctgtttacttgttggtttcttttcaatttcatccaatagagcttcagcttgataaagccaggtacttatgtgagccacgttcccatcaaatatttctagctggttctgatggttcatcaaggtattgcaccaatcttcagtccaggtacgaactcggctccacccagcgttaaggacgcagagcctctcttctaaaataggctcactgccctcaatcaagttttgcagggcagcactactctctgtgatggtatttaaatcagcttttctcttttccagatccttcagaacatttttagcccaggaaatttctgtatccaagtcaccaagcagaccttctgaagtggacttctgtaccaattcagtttcagtagcagaaagccattcagagagagaagcagcctctttcttcattttccgggccaactgtgatgctctttccagatcctgttttccttctgtcacctgtgcgcccaggtcattgtaaagaaccttcagggaagtcagctgctcatccatcccttttgggttgtccgtttgctgtttctggacaatatgtcttcctgttttaatcacagtttccacttcaagtttgacttcactcaaagttttatacagtttcatacacttgtccaggtgcgtctgtatgacgtcagggtctacgtccttcacatccagaacgtgaagttctgctttcacgccatccagcacacgcttgcagtccagcatgcgctgctcgaagttagctggcttctggaaaagctggaactttgtggacacctctcggagtttcctctgtagcacatccatctgacttcctcctctggcagtcctactctctggggaggtcaggggctgagaacgcatatttcttctcaactcctctagggttagctcatgggctgagatctctgcttggattttctgagcttcctgtggaacttggaaagcatctatcctgtcagtcaggtatgtggtgagctgtttgtccagctcccccaagctctcttgcaagacttgaagcatctggtcagtttcccgcagcacctggagttgcttttccaaagaaatctgcttgctctctgccaggtgacttagatcttcatatcggctgttgaaagcctccagtttctcactgattatatcatccaggatccccccatcaatcagagtctggccaagctctcgaatctgggtgcgattatctgccgggtggcgcagaacagattccagagactccagggcttcgttgacagcatccgtcttctcaggcaggacctctgtgctcttcatccgctcttccaaagtgtttaaccaggtagtttcaagatccaaatagtgaagcagttcaatccaacaagaccagacctcctctagcgtgtggcactttcctcgaattctattacaaagaagttggtaattctccagcacaacattcagctcagacgtcaactcctggccaccagagggcaccttggcagctaataacttgatgttgtccttgagaatcttcactctcacctccttctgcaacacatcctcttttgccctcttcatctcttccacagcactctcaagctcttctggtgacttgtactcaaaatcccgctccaaatattcttcctcggcctgggtcatccattcctgcatctctgccaagtctttcttcaggttcgcagctttttcttgactttcagacaacctacttttttgagtagcgatctccttgctaagtttctccagttgagtttggtagtcacctagtcttgtctgcacccaagtttttattccagcaactggaccacttcgaagattagtctctatttccttcatgtttttcagagatgattcaattgtttctatttcattaacaaatgcagagcactggtctaactgcctctgtagacctgcgtcgtctccttgggcagcctgctgtttcattaagaagtctttcacgccatccatccacttctcaatgactgttgaatcggcctcaaaagctctgagtgtgagagcaatttcctcaagcaaatgtagatctttggaaaccaagacctttagcttgttccactttccttgcacatcatcaaattcttgcttatataatttttctacatcaggatgaacatttttctccagagcctttgtttcttctgcaagtttatgtaatgcaggtttctgattctcaaggatttcatcaagggtctttttttcttgcagggccttctccaccttggcaagatcattaaggacattcagagacacctgggccttattttctgaatcatttagcacatctttcagtgttttcaatgtttccagatatgcatgtccaggttggcccttcagttcattctctagatgttgttgacgatcctctacagcctcttgtacagcttggtagcggcccagaaagctatcgaagccccgctggacaaaatctggggcagaaggctgagacatcagggccgagcagcttgcacgagccatttcaattttggggtgaaggccaagaagatttgtcaattcccgctgacaggaatccttcaagcttggcaaggactgccgggaagattcagaaatggaagtgtgttttacccactcctcctttgtcttgatgaccttttcaagctcatcaagctgcttgaaataagcatttatatcttcctgtagctgaatctttctttctagatcttccaaatgttgagatacattcttccattctgatgaaaccttctccagaacattttttatttcttcagtaggaaggccttttcccatttgctccacaaggatttgtccagtttggtttaattcatctgctctggggattctttctctctgttctttttctaatgccttcaacttctttttcatttcggaagtgtcttgcatcttcatatactcttttatctctgtggtctgaatggcagttttccatttcaaaatccagttcaacagctctgcacttatagcatcaaactttttcttagcttcaatatccacatggatctgtctcttctttgggggaggaggaggaggcagttcctgcttagatttttttgtaattgcttgttctcttacacgaacagtctccaaaaggtccttctgaggaatctgagacatccccagctttgctacagcctgagtcacctggttggaggaatcttctagtctctgaaccaaagaatcccatctttgagtcagttcctctgagtcactgttgatcttcttagatgccttggaattatcaagtaattgtcccacatcctggccaatctcactcagctgatccaatgtttgacgcttcatttccatgtcttccttcaaaatagccagacgtcgaacactgacacttagttccttttggtctttgaagttgcttgtctggactttatttaaagcctcttctttttcggttaaccaagctttcaacaagcactgttcttccaataattcctgccacaatatattgatttcttgtaacctattccagcgttcttcagtccaacggcatactgctgtccagcgctcaccaagtttctgtaactggtcttctaggatagctgtagcactctcaccactgttttcatcaacaatgaccaccatgtgagttagtgaatttactttcacctgttcagcctcaagatcactttgcaaacttttatgttcttctagcagcttttgtagagattttacatcatcatccagggggcaagtttccatcttctgaatgcgctcctctgtgagtgttaaccaggcggagagctgctgcagttgcttcttctgcagttccatcagcacatcgtgcagccgggactgtctgtccatactctccaccctaagagcctcccatctagcattcagcagggtcatctgttcctgaatctcaaattcttcttcgtctgacagagttccttgtgttatcagttggttgcctgcctgcaggacgctgcccacactgctctggtgtgcagtcagttccatcataaaagcttcatgggttgcaaactggtctttgacttcttcaacatcatcagaaatatcatcctgctcctggaaagtgtcctcagcagaaagcaaccaggtcagcacttcctccaacgcaatctgatagctgtccagatccatgtcaacctcagtgacagtgctgggagtttcagctcggggactctcatgctcctcctcaggcgctgtactctgtatattaattgcctcttcttcacattcttttttatatttccttgggagtgtctctacctcacggatggcgtctatggtgacttgctgaggtagcacctcaaacaaagatgttaaatacataattatggatttcttgtcaggaagctgaacggcaacatcttcaggatctaacagcttttcaattcccaaataagtttgagccttgctgaaggcatgttcaagtctctcaattggtgacattttgacaactttatcccagctgaagagatcaggtttatgtcggtggaggacagcattaaaggcgagtccatctgtccagctggtggtgaagttgaggacgttgacttggctgtagggcctggtggtctgacgcacccagctgagcaggatcttctcactgttcgtctgctgcaggtccgacatgacatccttcatgacatctttcacctgccagtgcaaaatgatgctccaaagtaaccccaaagtcagtttgtgatttccatccacaatgtcagttccccctatattcactaattccacattgttctgatgtaaaacctgcagcactctgttgacgttatttaaggcatgtacccttgtggaaccacgttcctttggcagtgatgttcctgtgaggccttctagaagatccaatagcttccttccatctttgaggtctgtgaacatatcattgatgggtggtttcccactctttgaaaatcgagcatttatccatttggtaaaggttttcttctgtacgtcattgtgttcatcaattaggttgagttggtgatgcaatccgatggcaggagattgcagctggggaatctggtctgaatgcggaatgaggagcaaagggccattatctctctctcctgtagtaggagagggcagatctggacttaatgatatcactgaattcgttctgcccattgtcaggactggcttcatgttctccatacttggccatcttgccagagtttcaagataatccaaaaactttaccaagtcctctttctaaggctttcaacttcctacgatggttcagcttgacatcaataccttgtcagttgcagcaagagatccccagagtccggaaaaggagagccggcgactgcgcgggactacacaccaatggggcgcccccctcctcctgtcccctca

SEQ ID NO: 10741 - RNA, 3965 nt, Homo sapiens
  source 1..3965: mol_type = other RNA
ctcatctgcaaagaagtaagtgggcaacgtcaaataaagttaaacggcatacacagggctgtagcttaaaccatatgtgtgtatatataagatatttgattgaaatttatgaatttattaatgtggccaaatcacggaaacaaatacatggatctatttgggatctagttggttatatggctgataaacatatggctgataaattataaataaccaaaacattgtggtaaaagagtcaaagaaaaaatgaagtaattgtgcaaggttaatatgaacagcagaaggaatgtaaaaatgtaaagtggtcttctaattcttatgtaagctttgtcatagttattaaaaagacggtatcatattagaaagcccccacccactttcccaatgctgtatacattatacaaatccgtgacaaatgtattaccatttccaaatacctctctgttcattaatttacacttgcatagaaagggaagaagaaaacaataatatatggttattataaaaacaaaatatccatttctctttggatagtcagtgttttactctttcagtagaacacacagtcagcactcaacatcgtgggccaaggagccatggagcttctgatttaatggaacttggaattggcatttgctgaaaagggcaacactgtacgtcaggaaacattggttggccggatgaatacttcacattgcctgtggcctgctgggaacatttgggcagcaagatggaaacgtgctgtgaatctgctccatgacctccgtgagatccgtgctggtgtcgtgcggtggggccagcaggtcctctcccgctgcctggtggaactgtgggccggaggcatctggatcaagcgagtagctcagtgcagaatgctgaggagaagcccatggggaaacaccattgattcgggaatcagattcaggctgctccagcagctgtcggaggcggtggagctgagactccagctgtttattgtgatcttctaaaatctgcatcctagcctccagccgacctttgtgctgcctgaggagttttgcttctgctataagttctgaatcctcagacgtgtgatggggagatataatcgactctggcggtgaaccgacagggagcccccttcggaggtgctggtccttcagctgctcatactccacctgtagatttctttgttcttcctccaggtcagcaatgatcctctccagttctccacgttcttccctctctactgacttcaggatctgagctgggctctgcggctggctcactggggactctcctccgagtgtttggcaatactgctggatgagggcgtgctcgtcttccacacttcctgtggtggagctgctatcagtgagaaaagacccattagtcctttccatctgggccagtcgtgtggcatattgttctattcttgaatgggtgtcatcatgaaacagttgaggagattgtgaggggtcatagtgctctggccacatactgatgagtgtgataggagtctctaagttgtcaccttcaagaactgtctggacaggcaggtaaccaagtcgagggtgtttggcaaagtacttcttcgacctgaacttgttcttaagtacctttgtgaagtctcgtacatcttccccagatgttgtaggtatacaatattccaccattgggtaatgtaatttgtgaccttttgctgttcgacccgaaaagaaacaactctggcagacatcatagttaaaatgcttaaggcttctatacctgaacccgacaattggacattctttacagatgttgcatttggcctgatgttttgcagtctccgctgctgccactcgatgtaaaactgggagccaaaccatggactgtggttccaaatgcatccaatctataaactctttcacacttatttctggtttattgttattctgttggaagcagctgcgaacactaggctcaatattactgcctccaaaagctgctacttcacctagctgccgggggatctggatggcatcatgaagtaacaggcccagctgcctctggtcacacatttctgttggccctgcaacttccttaaagagatatctgtatttttcttccaagagacctttggagagagacattaatccaatcttcagactctgcactctaatttttccagttcgacccgtgtcatagacattgagcaaccaattgagacacatatcaacacagagtggaacgttgaccaggtccttatgcatttgctcaagtccatcataagttgttgtcagacagttgatgacatctggaacactgaggagctggtcattttggttcaacttgtgctgtttgaaaatttcatttgttgtactcaactctaagagatccaaacatagtgctttttgtagtcttcggattttgattgctgtacggtaggcagaaaaacgtacattattcaggtcagcaagggattgaaagagttcggtcattttaggatggtcccaacaggtggtctgtgtttgatggttgatgtaatagggcactttattatgtgaaatggatctttgccacggcagctggactgacgtagagagaaaatgctgagaggatggtccaaaatctctgtgggcttcctgaagctgtttaaggcgatcatccacagaaacctgtaaaagtttccatcgcatattaaggtcatctagctggcgagacatctttagagagggatgcaggtcaagtggagacagctgactggataaatcattcaccgttttaactttaaagttgattggtgcaatttcttctctaaatgccatgattttttcaatgtgatcctgcagcgagtcaatgagtaagtctcccacgggcttccagccattccgcacggactctgcctccttcatgtcagcgtccaggtcatccatagctccctgcaggtctctgagtttctccaatgccttgtccacttgcttttgccaattgctagttacagcatttagactttcccatttttctttgacttcagaagactgtttgcgcatggctttggcaatcttttgggctctctcctcaggagttaattctgtttttgattgtaggtttcttcttggctcttcaggggcctcaattggctgatcagccaagaaaactcgggcctggtcgacagcattcaggacagaatattctttctcctttaactcccgtctcagggccttacaatggtcatactggagctgtaaggctggaacatctcctccaataggcatttgtttcttaagctcttcatctttcatattcagccatttgatcagttcttctaaggacatcagcaacctgttccacttctcagcgctggcctccaaatgggccctgatgctagcagattttgcttttaagtcattccatctttggttcatatcatccagtcgatgttgaagcatagtagcctcttcagaatttcccaaagcttttaccatcttctgcctgtttccgtcaatgcttttaaatatgtcattgtgggcatcaatttctgcctggatgtccttacagagcttctgataccgaggagaagaaactgccatcctttgtaagcgatgcaacaaaaccacaactttctgcagagacgttctcaccacagccatcattttaagtttaccacacttctggagacacctcagaatttgcattataaatgaagagcaacgatcatttcctcccggtcactggacaatgatttgtcagttctctgagcatgctcgtttccaggaaagcatttgaaagatacagggggttaggttctaggaaaaaggaggctggtattccttcaacttctcaatttaaaaaacacagacaaacgccacagagaaagccccccagcagatgctcacaggcagcacttgctcagcccggcatggccagaaatgaaggaagttgtcgagcagccaagcgctgccggctgcgggagaggagtgcgctcagtagccaaagaggatatt

SEQ ID NO: 10742 - RNA, 4426 nt, Homo sapiens
  source 1..4426: mol_type = other RNA
ctcatctgcaaagaagtaagtgggcaacgtcaaataaagttaaacggcatacacagggctgtagcttaaaccatatgtgtgtatatataagatatttgattgaaatttatgaatttattaatgtggccaaatcacggaaacaaatacatggatctatttgggatctagttggttatatggctgataaacatatggctgataaattataaataaccaaaacattgtggtaaaagagtcaaagaaaaaatgaagtaattgtgcaaggttaatatgaacagcagaaggaatgtaaaaatgtaaagtggtcttctaattcttatgtaagctttgtcatagttattaaaaagacggtatcatattagaaagcccccacccactttcccaatgctgtatacattatacaaatccgtgacaaatgtattaccatttccaaatacctctctgttcattaatttacacttgcatagaaagggaagaagaaaacaataatatatggttattataaaaacaaaatatccatttctctttggatagtcagtgttttactctttcagtagaacacacagtcagcactcaacatcgtgggccaaggagccatggagcttctgatttaatggaacttggaattggcatttgctgaaaagggcaacactgtacgtcaggaaacattggttggccggatgaatacttcacattgcctgtggcctgctgggaacatttgggcagcaagatggaaacgtgctgtgaatctgctccatgacctccgtgagatccgtgctggtgtcgtgcggtggggccagcaggtcctctcccgctgcctggtggaactgtgggccggaggcatctggatcaagcgagtagctcagtgcagaatgctgaggagaagcccatggggaaacaccattgattcgggaatcagattcaggctgctccagcagctgtcggaggcggtggagctgagactccagctgtttattgtgatcttctaaaatctgcatcctagcctccagccgacctttgtgctgcctgaggagttttgcttctgctataagttctgaatcctcagacgtgtgatggggagatataatcgactctggcggtgaaccgacagggagcccccttcggaggtgctggtccttcagctgctcatactccacctgtagatttctttgttcttcctccaggtcagcaatgatcctctccagttctccacgttcttccctctctactgacttcaggatctgagctgggctctgcggctggctcactggggactctcctccgagtgtttggcaatactgctggatgagggcgtgctcgtcttccacacttcctgtggtggagctgctatcagtgagaaaagacccattagtcctttccatctgggccagtcgtgtggcatattgttctattcttgaatgggtgtcatcatgaaacagttgaggagattgtgaggggtcatagtgctctggccacatactgatgagtgtgataggagtctctaagttgtcaccttcaagaactgtctggacaggcaggtaaccaagtcgagggtgtttggcaaagtacttcttcgacctgaacttgttcttaagtacctttgtgaagtctcgtacatcttccccagatgttgtaggtatacaatattccaccattgggtaatgtaatttgtgaccttttgctgttcgacccgaaaagaaacaactctggcagacatcatagttaaaatgcttaaggcttctatacctgaacccgacaattggacattctttacagatgttgcatttggcctgatgttttgcagtctccgctgctgccactcgatgtaaaactgggagccaaaccatggactgtggttccaaatgcatccaatctataaactctttcacacttatttctggtttattgttattctgttggaagcagctgcgaacactaggctcaatattactgcctccaaaagctgctacttcacctagctgccgggggatctggatggcatcatgaagtaacaggcccagctgcctctggtcacacatttctgttggccctgcaacttccttaaagagatatctgtatttttcttccaagagacctttggagagagacattaatccaatcttcagactctgcactctaatttttccagttcgacccgtgtcatagacattgagcaaccaattgagacacatatcaacacagagtggaacgttgaccaggtccttatgcatttgctcaagtccatcataagttgttgtcagacagttgatgacatctggaacactgaggagctggtcattttggttcaacttgtgctgtttgaaaatttcatttgttgtactcaactctaagagatccaaacatagtgctttttgtagtcttcggattttgattgctgtacggtaggcagaaaaacgtacattattcaggtcagcaagggattgaaagagttcggtcattttaggatggtcccaacaggtggtctgtgtttgatggttgatgtaatagggcactttattatgtgaaatggatctttgccacggcagctggactgacgtagagagaaaatgctgagaggatggtccaaaatctctgtgggcttcctgaagctgtttaaggcgatcatccacagaaacctgtaaaagtttccatcgcatattaaggtcatctagctggcgagacatctttagagagggatgcaggtcaagtggagacagctgactggataaatcattcaccgttttaactttaaagttgattggtgcaatttcttctctaaatgccatgattttttcaatgtgatcctgcagcgagtcaatgagtaagtctcccacgggcttccagccattccgcacggactctgcctccttcatgtcagcgtccaggtcatccatagctccctgcaggtctctgagtttctccaatgccttgtccacttgcttttgccaattgctagttacagcatttagactttcccatttttctttgacttcagaagactgtttgcgcatggctttggcaatcttttgggctctctcctcaggagttaattctgtttttgattgtaggtttcttcttggctcttcaggggcctcaattggctgatcagccaagaaaactcgggcctggtcgacagcattcaggacagaatattctttctcctttaactcccgtctcagggccttacaatggtcatactggagctgtaaggctggaacatctcctccaataggcatttgtttcttaagctcttcatctttcatattcagccatttgatcagttcttctaaggacatcagcaacctgttccacttctcagcgctggcctccaaatgggccctgatgctagcagattttgcttttaagtcattccatctttggttcatatcatccagtcgatgttgaagcatagtagcctcttcagaatttcccaaagcttttaccatcttctgcctgtttccgtcaatgcttttaaatatgtcattgtgggcatcaatttctgcctggatgtccttttcaaattttgtcagcagttcccgtaagttgaagttcagaccaatcattgtccagtagcccttgaagcctacatctttccggcaaacttccttcagacaacagcgtttaacttctaaacaccgtatcttttctggctatactttaaaatcctttgtaaaatcctttacaagccttgcccttgagctatggtccatcagcagcagcggcagcttgcgctgggacattttagccaccccactgtgggtccgttttttcatggacttcggagttcgcaaggaatagacctgcttctgtatttcctggtagctgtgttccacgaggctggcatggtctcctctttctctgggaagtccaggattcccttctgctcacctcactaatgacctgcaggccacaactgttctctccagggccccaagcttagagtttggtctcaattacatacagcaaaaaaagaagctatatcctggaaacttgcatgagagaagaaaaaaaaaaagccaagtattaccaacttcctccattcagaccgatttcagaacgaaaaaaaaaaaatcctgggtaaagagccagttttcaaagagcatgacttatgtagagttcgaaggaggagtgtactcttagctgaagaaacaccaaaacacaggacaagaggccaccggttctcactctcccagacaccagcagcctgggttgctatggtaaccaccaagctagtttcagtccatttccctaggtcagcctggcctaagggatgctgtcaatgcaacagaactaaacttgttttaaaaggtgttctgtctgtccagagaaaagctctcgcagcaaatctagtcccttctgccggctttgtggcaggggagagcagcctcagtgggctctggcagctcccctggctgatctgacagca

SEQ ID NO: 10743 - RNA, 2293 nt, Homo sapiens
  source 1..2293: mol_type = other RNA
ctcatttaagtagtctgatgcctgctctttctaacaaaccaatcatggcaaaaatttcaggctccctcccctgaattttgaaactacctaaaagcagaatgttttcccctggcaaatggttacttctttgaaaagtagacaatcttttttttttttttttaaatccaactaagccctttagaaagtactccagactacatgaggaggaagtgcaggagaactgacttcctattgtgccttgcataaaacattttgctaaaattaaaagcagctccaagtgcaaaagtaaatatttgtgcaaaaaggcacactgccaggtgcaatcttaaaacatcgtcaacttactcattttatagtgtttgactcttttaaataccagtcttttaaattatgaaacctagcaagtaaggggaaggaagttcacatcagaaaatacactttagaaaaggtacaagacattttgctggcaatttgctacttatttcataacatagatcaagtaagtgtttgttaaatattcacagtaatttcagagagaaacatatctccaaaacttcaacctattgcatttttaactatttttctgtacaatttataaaacatctgtcagtgtttttctgaataattccttcttgtcagtccttccctctctggatccagttataccttcaaggtgggttgtaggattcctttctcaatgagatgagtcttcagggttttatatatatttaactgctgttcaggttgaagcaccaacaactgctgtagcactttgctgggatttgggcccctgtctcaagactgcctttagaaagggtggaagtgagtaagtctgaagctggaaaagttctgagggctcacattctgtcacgaaggagtttacatcacttcggtattccactgggcagacaaagtactggtatttggataacacataggcagcaatgaatccaaacacaactgtggaaaagaaaccaccaatgaatccttcccaagtctttttaggagacaacttaattaatggagttctcccaaaaaaaaatccaaaaaggtaagcagttatgtcattgcagataacacttgatattggaacaaggaaccatatcatgccttcaaacagattttggatgacaaggtgtgactgagtgacagttatcagtaaagtgacatgagtccatgcgaacatataaaactgcagacgataatgtttcttcaccaaactcagtacaaacatgcagaaacctgccagatagagggcaaatgatataaatctatggtagcgaatgaggaactgaagttgttcttctctttgaacaaatgtagcaaaataatcagctacagtctctccatagaaaaagtagtttacacacaatagaaagtaccaacttagtgttctaaaccatggtagatcataagaatgatagactctataacctatagtgataatttcatggaagcatttcacttggatgcccagaacaagaagcatcagcatgaaggatcccatatagatgatcaggaaaaacaacgagatcatagttagagtgagaattccacgtatccaccagtttttccaccttgaagataaaccagatagagcttttttgagaatctcaggggttctatctgaggatggtggaatttccggaatatcagaatctgttctggaatccaaatctccatatctgtcatcaatatctgtttctttgtcgctggtgctctcggtttcgtggtcgccgccggccgcctctccctcgcggtgtggcggcgacaccgcttccctggggccggggcagcttccccggtgcctcagctccaacatcttccgctcccgcgctgccgtggcggcctcctcaagcaccccgaaacctgagctgcaagcagggttctgcaggcggggcgccccgccacctcgcagccgcgccctggagtcccgcggagccgcagccactaacgcggccccaccatagagcggccgccgcgccggtcacctccaaaacggcatcaacgagagagcgctcgaggccgcctgcagcgagcgcggctccggcggaggtcccgggcaggctccgggcgccaggcgcgagcagagaaggcggagacgcggcctccggttgccaggtgcgcgtctccacgcagaggcccaggtaggaggaggagaaggggcggggagaaaaggaggacgcttgacccgctttagcgcggctctgggctcccgccgccgcgcaggcccctcccgccccgccccccggagccggactcggagccggcttgtcccggccccgcacacttc

SEQ ID NO: 10744 - RNA, 2224 nt, Homo sapiens
  source 1..2224: mol_type = other RNA
ctcatttaagtagtctgatgcctgctctttctaacaaaccaatcatggcaaaaatttcaggctccctcccctgaattttgaaactacctaaaagcagaatgttttcccctggcaaatggttacttctttgaaaagtagacaatcttttttttttttttttaaatccaactaagccctttagaaagtactccagactacatgaggaggaagtgcaggagaactgacttcctattgtgccttgcataaaacattttgctaaaattaaaagcagctccaagtgcaaaagtaaatatttgtgcaaaaaggcacactgccaggtgcaatcttaaaacatcgtcaacttactcattttatagtgtttgactcttttaaataccagtcttttaaattatgaaacctagcaagtaaggggaaggaagttcacatcagaaaatacactttagaaaaggtacaagacattttgctggcaatttgctacttatttcataacatagatcaagtaagtgtttgttaaatattcacagtaatttcagagagaaacatatctccaaaacttcaacctattgcatttttaactatttttctgtacaatttataaaacatctgtcagtgtttttctgaataattccttcttgtcagtccttccctctctggatccagttataccttcaaggtgggttgtaggattcctttctcaatgagatgagtcttcagggttttatatatatttaactgctgttcaggttgaagcaccaacaactgctgtagcactttgctgggatttgggcccctgtctcaagactgcctttagaaagggtggaagtgagtaagtctgaagctggaaaagttctgagggctcacattctgtcacgaaggagtttacatcacttcggtattccactgggcagacaaagtactggtatttggataacacataggcagccttaattaatggagttctcccaaaaaaaaatccaaaaaggtaagcagttatgtcattgcagataacacttgatattggaacaaggaaccatatcatgccttcaaacagattttggatgacaaggtgtgactgagtgacagttatcagtaaagtgacatgagtccatgcgaacatataaaactgcagacgataatgtttcttcaccaaactcagtacaaacatgcagaaacctgccagatagagggcaaatgatataaatctatggtagcgaatgaggaactgaagttgttcttctctttgaacaaatgtagcaaaataatcagctacagtctctccatagaaaaagtagtttacacacaatagaaagtaccaacttagtgttctaaaccatggtagatcataagaatgatagactctataacctatagtgataatttcatggaagcatttcacttggatgcccagaacaagaagcatcagcatgaaggatcccatatagatgatcaggaaaaacaacgagatcatagttagagtgagaattccacgtatccaccagtttttccaccttgaagataaaccagatagagcttttttgagaatctcaggggttctatctgaggatggtggaatttccggaatatcagaatctgttctggaatccaaatctccatatctgtcatcaatatctgtttctttgtcgctggtgctctcggtttcgtggtcgccgccggccgcctctccctcgcggtgtggcggcgacaccgcttccctggggccggggcagcttccccggtgcctcagctccaacatcttccgctcccgcgctgccgtggcggcctcctcaagcaccccgaaacctgagctgcaagcagggttctgcaggcggggcgccccgccacctcgcagccgcgccctggagtcccgcggagccgcagccactaacgcggccccaccatagagcggccgccgcgccggtcacctccaaaacggcatcaacgagagagcgctcgaggccgcctgcagcgagcgcggctccggcggaggtcccgggcaggctccgggcgccaggcgcgagcagagaaggcggagacgcggcctccggttgccaggtgcgcgtctccacgcagaggcccaggtaggaggaggagaaggggcggggagaaaaggaggacgcttgacccgctttagcgcggctctgggctcccgccgccgcgcaggcccctcccgccccgccccccggagccggactcggagccggcttgtcccggccccgcacacttc

SEQ ID NO: 10745 - RNA, 2397 nt, Homo sapiens
  source 1..2397: mol_type = other RNA
ctcatttaagtagtctgatgcctgctctttctaacaaaccaatcatggcaaaaatttcaggctccctcccctgaattttgaaactacctaaaagcagaatgttttcccctggcaaatggttacttctttgaaaagtagacaatcttttttttttttttttaaatccaactaagccctttagaaagtactccagactacatgaggaggaagtgcaggagaactgacttcctattgtgccttgcataaaacattttgctaaaattaaaagcagctccaagtgcaaaagtaaatatttgtgcaaaaaggcacactgccaggtgcaatcttaaaacatcgtcaacttactcattttatagtgtttgactcttttaaataccagtcttttaaattatgaaacctagcaagtaaggggaaggaagttcacatcagaaaatacactttagaaaaggtacaagacattttgctggcaatttgctacttatttcataacatagatcaagtaagtgtttgttaaatattcacagtaatttcagagagaaacatatctccaaaacttcaacctattgcatttttaactatttttctgtacaatttataaaacatctgtcagtgtttttctgaataattccttcttgtcagtccttccctctctggatccagttataccttcaaggtgggttgtaggattcctttctcaatgagatgagtcttcagggttttatatatatttaactgctgttcaggttgaagcaccaacaactgctgtagcactttgctgggatttgggccccttataaaacttgtgatgtacacatgtacaaaagttgccatcaaatactgacaatcaaatctgtccattatcccaccatgtccaggaatggtatttgcaaaatcctgtctcaagactgcctttagaaagggtggaagtgagtaagtctgaagctggaaaagttctgagggctcacattctgtcacgaaggagtttacatcacttcggtattccactgggcagacaaagtactggtatttggataacacataggcagcaatgaatccaaacacaactgtggaaaagaaaccaccaatgaatccttcccaagtctttttaggagacaacttaattaatggagttctcccaaaaaaaaatccaaaaaggtaagcagttatgtcattgcagataacacttgatattggaacaaggaaccatatcatgccttcaaacagattttggatgacaaggtgtgactgagtgacagttatcagtaaagtgacatgagtccatgcgaacatataaaactgcagacgataatgtttcttcaccaaactcagtacaaacatgcagaaacctgccagatagagggcaaatgatataaatctatggtagcgaatgaggaactgaagttgttcttctctttgaacaaatgtagcaaaataatcagctacagtctctccatagaaaaagtagtttacacacaatagaaagtaccaacttagtgttctaaaccatggtagatcataagaatgatagactctataacctatagtgataatttcatggaagcatttcacttggatgcccagaacaagaagcatcagcatgaaggatcccatatagatgatcaggaaaaacaacgagatcatagttagagtgagaattccacgtatccaccagtttttccaccttgaagataaaccagatagagcttttttgagaatctcaggggttctatctgaggatggtggaatttccggaatatcagaatctgttctggaatccaaatctccatatctgtcatcaatatctgtttctttgtcgctggtgctctcggtttcgtggtcgccgccggccgcctctccctcgcggtgtggcggcgacaccgcttccctggggccggggcagcttccccggtgcctcagctccaacatcttccgctcccgcgctgccgtggcggcctcctcaagcaccccgaaacctgagctgcaagcagggttctgcaggcggggcgccccgccacctcgcagccgcgccctggagtcccgcggagccgcagccactaacgcggccccaccatagagcggccgccgcgccggtcacctccaaaacggcatcaacgagagagcgctcgaggccgcctgcagcgagcgcggctccggcggaggtcccgggcaggctccgggcgccaggcgcgagcagagaaggcggagacgcggcctccggttgccaggtgcgcgtctccacgcagaggcccaggtaggaggaggagaaggggcggggagaaaaggaggacgcttgacccgctttagcgcggctctgggctcccgccgccgcgcaggcccctcccgccccgccccccggagccggactcggagccggcttgtcccggccccgcacacttc

SEQ ID NO: 10746 - RNA, 2328 nt, Homo sapiens
  source 1..2328: mol_type = other RNA
ctcatttaagtagtctgatgcctgctctttctaacaaaccaatcatggcaaaaatttcaggctccctcccctgaattttgaaactacctaaaagcagaatgttttcccctggcaaatggttacttctttgaaaagtagacaatcttttttttttttttttaaatccaactaagccctttagaaagtactccagactacatgaggaggaagtgcaggagaactgacttcctattgtgccttgcataaaacattttgctaaaattaaaagcagctccaagtgcaaaagtaaatatttgtgcaaaaaggcacactgccaggtgcaatcttaaaacatcgtcaacttactcattttatagtgtttgactcttttaaataccagtcttttaaattatgaaacctagcaagtaaggggaaggaagttcacatcagaaaatacactttagaaaaggtacaagacattttgctggcaatttgctacttatttcataacatagatcaagtaagtgtttgttaaatattcacagtaatttcagagagaaacatatctccaaaacttcaacctattgcatttttaactatttttctgtacaatttataaaacatctgtcagtgtttttctgaataattccttcttgtcagtccttccctctctggatccagttataccttcaaggtgggttgtaggattcctttctcaatgagatgagtcttcagggttttatatatatttaactgctgttcaggttgaagcaccaacaactgctgtagcactttgctgggatttgggccccttataaaacttgtgatgtacacatgtacaaaagttgccatcaaatactgacaatcaaatctgtccattatcccaccatgtccaggaatggtatttgcaaaatcctgtctcaagactgcctttagaaagggtggaagtgagtaagtctgaagctggaaaagttctgagggctcacattctgtcacgaaggagtttacatcacttcggtattccactgggcagacaaagtactggtatttggataacacataggcagccttaattaatggagttctcccaaaaaaaaatccaaaaaggtaagcagttatgtcattgcagataacacttgatattggaacaaggaaccatatcatgccttcaaacagattttggatgacaaggtgtgactgagtgacagttatcagtaaagtgacatgagtccatgcgaacatataaaactgcagacgataatgtttcttcaccaaactcagtacaaacatgcagaaacctgccagatagagggcaaatgatataaatctatggtagcgaatgaggaactgaagttgttcttctctttgaacaaatgtagcaaaataatcagctacagtctctccatagaaaaagtagtttacacacaatagaaagtaccaacttagtgttctaaaccatggtagatcataagaatgatagactctataacctatagtgataatttcatggaagcatttcacttggatgcccagaacaagaagcatcagcatgaaggatcccatatagatgatcaggaaaaacaacgagatcatagttagagtgagaattccacgtatccaccagtttttccaccttgaagataaaccagatagagcttttttgagaatctcaggggttctatctgaggatggtggaatttccggaatatcagaatctgttctggaatccaaatctccatatctgtcatcaatatctgtttctttgtcgctggtgctctcggtttcgtggtcgccgccggccgcctctccctcgcggtgtggcggcgacaccgcttccctggggccggggcagcttccccggtgcctcagctccaacatcttccgctcccgcgctgccgtggcggcctcctcaagcaccccgaaacctgagctgcaagcagggttctgcaggcggggcgccccgccacctcgcagccgcgccctggagtcccgcggagccgcagccactaacgcggccccaccatagagcggccgccgcgccggtcacctccaaaacggcatcaacgagagagcgctcgaggccgcctgcagcgagcgcggctccggcggaggtcccgggcaggctccgggcgccaggcgcgagcagagaaggcggagacgcggcctccggttgccaggtgcgcgtctccacgcagaggcccaggtaggaggaggagaaggggcggggagaaaaggaggacgcttgacccgctttagcgcggctctgggctcccgccgccgcgcaggcccctcccgccccgccccccggagccggactcggagccggcttgtcccggccccgcacacttc

SEQ ID NO: 10747 - RNA, 2321 nt, Homo sapiens
  source 1..2321: mol_type = other RNA
ctcatttaagtagtctgatgcctgctctttctaacaaaccaatcatggcaaaaatttcaggctccctcccctgaattttgaaactacctaaaagcagaatgttttcccctggcaaatggttacttctttgaaaagtagacaatcttttttttttttttttaaatccaactaagccctttagaaagtactccagactacatgaggaggaagtgcaggagaactgacttcctattgtgccttgcataaaacattttgctaaaattaaaagcagctccaagtgcaaaagtaaatatttgtgcaaaaaggcacactgccaggtgcaatcttaaaacatcgtcaacttactcattttatagtgtttgactcttttaaataccagtcttttaaattatgaaacctagcaagtaaggggaaggaagttcacatcagaaaatacactttagaaaaggtacaagacattttgctggcaatttgctacttatttcataacatagatcaagtaagtgtttgttaaatattcacagtaatttcagagagaaacatatctccaaaacttcaacctattgcatttttaactatttttctgtacaatttataaaacatctgtcagtgtttttctgaataattccttcttgtcagtccttccctctctggatccagttataccttcaaggtgggttgtaggattcctttctcaatgagatgagtcttcagggttttatatatatttaactgctgttcaggttgaagcaccaacaactgctgtagcactttgctgggatttgggccccttataaaacttgtgatgtacacatgtacaaaagttgccatcaaatactgacaatcaaatctgtccattatcccaccatgtccaggaatggtatttgcaaaatccttgattttgaaggctcttttgaatccactagcaaagaagcctccaaatgggccaattaaagatgcaaaggttgacagtgcaatgctgtggatctggaaagggtacaagctcactctttcctgtctcaagactgcctttagaaagggtggaagtgagtaagtctgaagctggaaaagttctgagggctcacattctgtcacgaaggagtttacatcacttcggtattccactgggcagacaaagtactggtatttggataacacataggcagcaatgaatccaaacacaactgtggaaaagaaaccaccaatgaatccttcccaagtctttttaggagacaacttaattaatggagttctcccaaaaaaaaatccaaaaaggtaagcagttatgtcattgcagataacacttgatattggaacaaggaaccatatcatgccttcaaacagattttggatgacaaggtgtgactgagtgacagttatcagtaaagtgacatgagtccatgcgaacatataaaactgcagacgataatgtttcttcaccaaactcagtacaaacatgcagaaacctgccagatagagggcaaatgatataaatctatggtagcgaatgaggaactgaagttgttcttctctttgaacaaatgtagcaaaataatcagctacagtctctccatagaaaaagtagtttacacacaatagaaagtaccaacttagtgttctaaaccatggtagatcataagaatgatagactctataacctatagtgataatttcatggaagcatttcacttggatgcccagaacaagaagcatcagcatgaaggatcccatatagatgatcaggaaaaacaacgagatcatagttagagtgagaattccacgtatccaccagtttttccaccttgaagataaaccagatagagcttttttgagaatctcaggggttctatctgaggatggtggaatttccggaatatcagaatctgttctggaatccaaatctccatatctgtcatcaatatctgtttctttgtcgctggtgctctcggtttcgtggtcgccgccggccgcctctccctcgcggtgtggcggcgacaccgcttccctggggccggggcagcttccccggtgcctcagctccaacatcttccgctcccgcgctgccgtggcggcctcctcaagcaccccgaaacctgagctgcaagcagggttctgcaggcggggcgccccgccacctcgcagccgcgccctggagtcccgcggagccgcagccactaacgcggccccaccatagagcggccgccgcgccggtcacctccaaaacggcatcaacgagagagcgctcgaggccgcctgcagcgagcgcggctccggcggaggtcccgggcaggctccgggcgccaggcgcgagcagagaaggc

SEQ ID NO: 10748 - RNA, 2448 nt, Homo sapiens
  source 1..2448: mol_type = other RNA
ctcatttaagtagtctgatgcctgctctttctaacaaaccaatcatggcaaaaatttcaggctccctcccctgaattttgaaactacctaaaagcagaatgttttcccctggcaaatggttacttctttgaaaagtagacaatcttttttttttttttttaaatccaactaagccctttagaaagtactccagactacatgaggaggaagtgcaggagaactgacttcctattgtgccttgcataaaacattttgctaaaattaaaagcagctccaagtgcaaaagtaaatatttgtgcaaaaaggcacactgccaggtgcaatcttaaaacatcgtcaacttactcattttatagtgtttgactcttttaaataccagtcttttaaattatgaaacctagcaagtaaggggaaggaagttcacatcagaaaatacactttagaaaaggtacaagacattttgctggcaatttgctacttatttcataacatagatcaagtaagtgtttgttaaatattcacagtaatttcagagagaaacatatctccaaaacttcaacctattgcatttttaactatttttctgtacaatttataaaacatctgtcagtgtttttctgaataattccttcttgtcagtccttccctctctggatccagttataccttcaaggtgggttgtaggattcctttctcaatgagatgagtcttcagggttttatatatatttaactgctgttcaggttgaagcaccaacaactgctgtagcactttgctgggatttgggccccttataaaacttgtgatgtacacatgtacaaaagttgccatcaaatactgacaatcaaatctgtccattatcccaccatgtccaggaatggtatttgcaaaatccttgattttgaaggctcttttgaatccactagcaaagaagcctccaaatgggccaattaaagatgcaaaggttgacagtgcaatgctgtggatctggaaagggtacaagctcactctttcctgtctcaagactgcctttagaaagggtggaagtgagtaagtctgaagctggaaaagttctgagggctcacattctgtcacgaaggagtttacatcacttcggtattccactgggcagacaaagtactggtatttggataacacataggcagccttaattaatggagttctcccaaaaaaaaatccaaaaaggtaagcagttatgtcattgcagataacacttgatattggaacaaggaaccatatcatgccttcaaacagattttggatgacaaggtgtgactgagtgacagttatcagtaaagtgacatgagtccatgcgaacatataaaactgcagacgataatgtttcttcaccaaactcagtacaaacatgcagaaacctgccagatagagggcaaatgatataaatctatggtagcgaatgaggaactgaagttgttcttctctttgaacaaatgtagcaaaataatcagctacagtctctccatagaaaaagtagtttacacacaatagaaagtaccaacttagtgttctaaaccatggtagatcataagaatgatagactctataacctatagtgataatttcatggaagcatttcacttggatgcccagaacaagaagcatcagcatgaaggatcccatatagatgatcaggaaaaacaacgagatcatagttagagtgagaattccacgtatccaccagtttttccaccttgaagataaaccagatagagcttttttgagaatctcaggggttctatctgaggatggtggaatttccggaatatcagaatctgttctggaatccaaatctccatatctgtcatcaatatctgtttctttgtcgctggtgctctcggtttcgtggtcgccgccggccgcctctccctcgcggtgtggcggcgacaccgcttccctggggccggggcagcttccccggtgcctcagctccaacatcttccgctcccgcgctgccgtggcggcctcctcaagcaccccgaaacctgagctgcaagcagggttctgcaggcggggcgccccgccacctcgcagccgcgccctggagtcccgcggagccgcagccactaacgcggccccaccatagagcggccgccgcgccggtcacctccaaaacggcatcaacgagagagcgctcgaggccgcctgcagcgagcgcggctccggcggaggtcccgggcaggctccgggcgccaggcgcgagcagagaaggcggagacgcggcctccggttgccaggtgcgcgtctccacgcagaggcccaggtaggaggaggagaaggggcggggagaaaaggaggacgcttgacccgctttagcgcggctctgggctcccgccgccgcgcaggcccctcccgccccgccccccggagccggactcggagccggcttgtcccggccccgcacacttc

SEQ ID NO: 10749 - RNA, 3739 nt, Homo sapiens
  source 1..3739: mol_type = other RNA
ctcccacttccagatctttctgtacctgtgtgtttgggctcctactcccacctctcccaggcgcagggagaggacaaaaagcataagggactctgttcaacccagcaaaagtcagtttcccagtggagaggcaaagccccacccagaacataaacatgcatgggaccaaggttagtgcccagacaggacagacttgcacagaacaagagggcacagtgggatccatgcggcaattacaggagcttccagcactaacagaggagccttatcccaccttcatcacacacacttagatggacacacacacactctcgctcacactctcacacatgtgcacacatacacacactctctctctctgcagccacactcaaatctgctaaactcctacaacctcccccagcaggtcatttgacaattctgcatcttccgctctctggtgctggggctctggtcagaggcgagccaatgtcttatcattagagagatgtgggattaggtaaggggcagagtcatggcactgctcacacaccttcccgaaactggggtctattcagttttttgacaagatcaaaagcaattcttaactggtcattatttttttttaaggtaattagaacactattgtttatacaatattgaaaaaatacaattttttattgtttgaactcaaatcaccacccagcactttaagcctaccctaaatagcacctacaataaatgtcatagcacaagcaaactgcaaagtcagcaggtaagcaagttagacagtgccagcagagagaccctccctcccccaaagcaatgagaagacagcgtgctaggtaagagtgaagtacaccattacatgttaaatagttaatactacccttccagcaagccacagatgctagatggataactcagtacggttaactaaccacagccctacatcactgcacttttttttttttttaaagaaaaccttttgcttcatgcccgtaattaacataaagtaagtaaattctttgtctttttatttaggaaaataatcatgctaaaagcaagttgtactttatatagattttcaaacaaaagattgattgtgctttttgaataaaaaagatagggtatcttccaacctcactgacttaaaccttgtggaatacagcacttctaaactaaaaacacacgtcaaaaagaaaaattaaataatcccagtgggatgctcaaaaatcgtctttagaaggttttaggattggctaattctgctattatcttattggctgcggcaaaaaaagaacacagagctgctgtctaaaatttctccaaactcccctccgagttcagcaggcaacactcagatttgaaagaaactctgcagcaacctggacatatggttagctgagtcgacatttgattagcaggcattttaaactgatttcctcttaacatacgcaggagagaaaacattttcttcctgcagggcatgttctactacatcatatttctgaatcccttcttcctattcggtcactctctgaaaaaagctggtttgtttttcccatgtagaatcactctgggtacaagaacctttatttgttccaattattatttgttttaaatttagaacctgtgttgggtctaaaatacccatttcccactcccacaagcagatgatgaccaggctgctgccaagagcagcagaaaaagggaaaaccaaaccagaacatgaaggcaagtacccagggctttgcagtcaccacgtgggtcgtcttctcaagtctaatggtccatgagcggcttgtccaaggaggcggccgcctcttggtaggtgaagatgaaatctgcaacctttctaagcacaatacacacacacacacaccaaaaaaataacccccccagaaacacaaccctcatatttaaagctcttaagttcagggtagcggtctcaaactgccaaacactaggatgaggatgtgactctgcatgtgttttggatgagaggaagcatcgtcccagtcacttttctcctcctgtgctgtcctttcaaaaacaggtctggatttcacgctctaccccaagaaaaagaactggttcagaaaacacttccccaagtttctccaacagaacactgtggctgcagggcctggtagtgtgaagggcagcaactgacatataaaaatgtacttaaaatcagagtcaaaaaatggttttaagttttaatactcttaattagctccctgctttatactgtaactccacagaagacatagggccacctaggattcacaggaaggagcagctctgattcttacatggctggctccgatgcccccacagcaggcctcttcctccccaagtttttcctctccatttcaaaaaagcactattttatcttcacatccaagagctggttggtttggtttgtttctttggaaaccaataaaagaagcaattttttcctgttctttttactcacatctacctatcagagcggctatttccttcgacagttcagtagcacacaggctgacttggccacatggactcatgaatgcatgcattcagaccgcatattgctaccaaatggaatgtgggaatatgctatgcacctcaggttgagaaatgaccaagaaatcaagatctaaagggtgatatataatatatatatatcaatgctattattcataaaaaccttgtttagtaataaaaaaaattgctttgtttaaatatgaatattatagtctgcttctcatggttaggaaataatagtctttctgaaaagcaggtgctttttctactacaactccatatcctgggcctcatcttcggaaaagtcagacatagagctctccgatgagctgtccccggtaccctcttcctgttctttcagcgcctcctccgtggcgtatttctggatgtactctttaattttctgcttgtattcttctggtcggtggaggtacatggctgcagcgtcaccattgagaggatctatggggttaggataggccaataactgaggcaggaaggactcaaatatattggtaagatcatagagagctgtccaagtttgattaattacatctagacacacagttcctgacgcttcatcaatgttgggatggaaaattttattcatgaatcctatagatggagatttgaaagggtatttatcaggtaggtccactctaactttccatactccgccttcatatggtgttccttgtggtccataaaacttcactacaaattcattaagtcctcccaggatcgtaacctcatgtttactctcgatgagcttgaccacgtccgtgtccatccgcctcttgcccggactgggagatgacatggtgtcgccgccgcctctctcccttcctcggcccgtctgtcacgggcccggggccccggctctgaggagcccgcggccgcgccggctcctcggtggaggtggcaacacccccgcggtcccggcggtcccgtcagccgccgccgccgccccccgcacgggggaacaccgggcactgtccggccgggtgggggtggggaccctgcggcgcccggctcgggctgcccctctccggctgtggttccgccgcggccctgccccggcgctcctctgcgccgcgcgacgctccctcctgcctgctgtggctcgctcgcctgctccccactcaccctctgaccggctcctagcagcctccactataagcggacgactcctgctcagtcggcctccctaccccagcctcgctct

SEQ ID NO: 10750 - RNA, 3360 nt, Homo sapiens
  source 1..3360: mol_type = other RNA
ctcccacttccagatctttctgtacctgtgtgtttgggctcctactcccacctctcccaggcgcagggagaggacaaaaagcataagggactctgttcaacccagcaaaagtcagtttcccagtggagaggcaaagccccacccagaacataaacatgcatgggaccaaggttagtgcccagacaggacagacttgcacagaacaagagggcacagtgggatccatgcggcaattacaggagcttccagcactaacagaggagccttatcccaccttcatcacacacacttagatggacacacacacactctcgctcacactctcacacatgtgcacacatacacacactctctctctctgcagccacactcaaatctgctaaactcctacaacctcccccagcaggtcatttgacaattctgcatcttccgctctctggtgctggggctctggtcagaggcgagccaatgtcttatcattagagagatgtgggattaggtaaggggcagagtcatggcactgctcacacaccttcccgaaactggggtctattcagttttttgacaagatcaaaagcaattcttaactggtcattatttttttttaaggtaattagaacactattgtttatacaatattgaaaaaatacaattttttattgtttgaactcaaatcaccacccagcactttaagcctaccctaaatagcacctacaataaatgtcatagcacaagcaaactgcaaagtcagcaggtaagcaagttagacagtgccagcagagagaccctccctcccccaaagcaatgagaagacagcgtgctaggtaagagtgaagtacaccattacatgttaaatagttaatactacccttccagcaagccacagatgctagatggataactcagtacggttaactaaccacagccctacatcactgcacttttttttttttttaaagaaaaccttttgcttcatgcccgtaattaacataaagtaagtaaattctttgtctttttatttaggaaaataatcatgctaaaagcaagttgtactttatatagattttcaaacaaaagattgattgtgctttttgaataaaaaagatagggtatcttccaacctcactgacttaaaccttgtggaatacagcacttctaaactaaaaacacacgtcaaaaagaaaaattaaataatcccagtgggatgctcaaaaatcgtctttagaaggttttaggattggctaattctgctattatcttattggctgcggcaaaaaaagaacacagagctgctgtctaaaatttctccaaactcccctccgagttcagcaggcaacactcagatttgaaagaaactctgcagcaacctggacatatggttagctgagtcgacatttgattagcaggcattttaaactgatttcctcttaacatacgcaggagagaaaacattttcttcctgcagggcatgttctactacatcatatttctgaatcccttcttcctattcggtcactctctgaaaaaagctggtttgtttttcccatgtagaatcactctgggtacaagaacctttatttgttccaattattatttgttttaaatttagaacctgtgttgggtctaaaatacccatttcccactcccacaagcagatgatgaccaggctgctgccaagagcagcagaaaaagggaaaaccaaaccagaacatgaaggcaagtacccagggctttgcagtcaccacgtgggtcgtcttctcaagtctaatggtccatgagcggcttgtccaaggaggcggccgcctcttggtaggtgaagatgaaatctgcaacctttctaagcacaatacacacacacacacaccaaaaaaataacccccccagaaacacaaccctcatatttaaagctcttaagttcagggtagcggtctcaaactgccaaacactaggatgaggatgtgactctgcatgtgttttggatgagaggaagcatcgtcccagtcacttttctcctcctgtgctgtcctttcaaaaacaggtctggatttcacgctctaccccaagaaaaagaactggttcagaaaacacttccccaagtttctccaacagaacactgtggctgcagggcctggtagtgtgaagggcagcaactgacatataaaaatgtacttaaaatcagagtcaaaaaatggttttaagttttaatactcttaattagctccctgctttatactgtaactccacagaagacatagggccacctaggattcacaggaaggagcagctctgattcttacatggctggctccgatgcccccacagcaggcctcttcctccccaagtttttcctctccatttcaaaaaagcactattttatcttcacatccaagagctggttggtttggtttgtttctttggaaaccaataaaagaagcaattttttcctgttctttttactcacatctacctatcagagcggctatttccttcgacagttcagtagcacacaggctgacttggccacatggactcatgaatgcatgcattcagaccgcatattgctaccaaatggaatgtgggaatatgctatgcacctcaggttgagaaatgaccaagaaatcaagatctaaagggtgatatataatatatatatatcaatgctattattcataaaaaccttgtttagtaataaaaaaaattgctttgtttaaatatgaatattatagtctgcttctcatggttaggaaataatagtctttctgaaaagcaggtgctttttctactacaactccatatcctgggcctcatcttcggaaaagtcagacatagagctctccgatgagctgtccccggtaccctcttcctgttctttcagcgcctcctccgtggcgtatttctggatgtactctttaattttctgcttgtattcttctggtcggtggaggtacatggctgcagcgtcaccattgagaggatctatggggttaggataggccaataactgaggcaggaaggactcaaatatattggtaagatcatagagagctgtccaagtttgattaattacatctagacacacagttcctgacgcttcatcaatgttgggatggaaaattttattcatgaatcctatagatggagatttgaaagggtatttatcaggtaggtccactctaactttccatactccgccttcatatggtgttccttgtggtccataaaacttcactacaaattcattaagtcctcccaggatcgtaacctcatgtttactctcgatgcctctgaccggctcctagcagcctccactataagcggacgactcctgctcagtcggcctccctaccccagcctcgctct

SEQ ID NO: 10751 - RNA, 3646 nt, Homo sapiens
  source 1..3646: mol_type = other RNA
ctcccacttccagatctttctgtacctgtgtgtttgggctcctactcccacctctcccaggcgcagggagaggacaaaaagcataagggactctgttcaacccagcaaaagtcagtttcccagtggagaggcaaagccccacccagaacataaacatgcatgggaccaaggttagtgcccagacaggacagacttgcacagaacaagagggcacagtgggatccatgcggcaattacaggagcttccagcactaacagaggagccttatcccaccttcatcacacacacttagatggacacacacacactctcgctcacactctcacacatgtgcacacatacacacactctctctctctgcagccacactcaaatctgctaaactcctacaacctcccccagcaggtcatttgacaattctgcatcttccgctctctggtgctggggctctggtcagaggcgagccaatgtcttatcattagagagatgtgggattaggtaaggggcagagtcatggcactgctcacacaccttcccgaaactggggtctattcagttttttgacaagatcaaaagcaattcttaactggtcattatttttttttaaggtaattagaacactattgtttatacaatattgaaaaaatacaattttttattgtttgaactcaaatcaccacccagcactttaagcctaccctaaatagcacctacaataaatgtcatagcacaagcaaactgcaaagtcagcaggtaagcaagttagacagtgccagcagagagaccctccctcccccaaagcaatgagaagacagcgtgctaggtaagagtgaagtacaccattacatgttaaatagttaatactacccttccagcaagccacagatgctagatggataactcagtacggttaactaaccacagccctacatcactgcacttttttttttttttaaagaaaaccttttgcttcatgcccgtaattaacataaagtaagtaaattctttgtctttttatttaggaaaataatcatgctaaaagcaagttgtactttatatagattttcaaacaaaagattgattgtgctttttgaataaaaaagatagggtatcttccaacctcactgacttaaaccttgtggaatacagcacttctaaactaaaaacacacgtcaaaaagaaaaattaaataatcccagtgggatgctcaaaaatcgtctttagaaggttttaggattggctaattctgctattatcttattggctgcggcaaaaaaagaacacagagctgctgtctaaaatttctccaaactcccctccgagttcagcaggcaacactcagatttgaaagaaactctgcagcaacctggacatatggttagctgagtcgacatttgattagcaggcattttaaactgatttcctcttaacatacgcaggagagaaaacattttcttcctgcagggcatgttctactacatcatatttctgaatcccttcttcctattcggtcactctctgaaaaaagctggtttgtttttcccatgtagaatcactctgggtacaagaacctttatttgttccaattattatttgttttaaatttagaacctgtgttgggtctaaaatacccatttcccactcccacaagcagatgatgaccaggctgctgccaagagcagcagaaaaagggaaaaccaaaccagaacatgaaggcaagtacccagggctttgcagtcaccacgtgggtcgtcttctcaagtctaatggtccatgagcggcttgtccaaggaggcggccgcctcttggtaggtgaagatgaaatctgcaacctttctaagcacaatacacacacacacacaccaaaaaaataacccccccagaaacacaaccctcatatttaaagctcttaagttcagggtagcggtctcaaactgccaaacactaggatgaggatgtgactctgcatgtgttttggatgagaggaagcatcgtcccagtcacttttctcctcctgtgctgtcctttcaaaaacaggtctggatttcacgctctaccccaagaaaaagaactggttcagaaaacacttccccaagtttctccaacagaacactgtggctgcagggcctggtagtgtgaagggcagcaactgacatataaaaatgtacttaaaatcagagtcaaaaaatggttttaagttttaatactcttaattagctccctgctttatactgtaactccacagaagacatagggccacctaggattcacaggaaggagcagctctgattcttacatggctggctccgatgcccccacagcaggcctcttcctccccaagtttttcctctccatttcaaaaaagcactattttatcttcacatccaagagctggttggtttggtttgtttctttggaaaccaataaaagaagcaattttttcctgttctttttactcacatctacctatcagagcggctatttccttcgacagttcagtagcacacaggctgacttggccacatggactcatgaatgcatgcattcagaccgcatattgctaccaaatggaatgtgggaatatgctatgcacctcaggttgagaaatgaccaagaaatcaagatctaaagggtgatatataatatatatatatcaatgctattattcataaaaaccttgtttagtaataaaaaaaattgctttgtttaaatatgaatattatagtctgcttctcatggttaggaaataatagtctttctgaaaagcaggtgctttttctactacaactccatatcctgggcctcatcttcggaaaagtcagacatagagctctccgatgagctgtccccggtaccctcttcctgttctttcagcgcctcctccgtggcgtatttctggatgtactctttaattttctgcttgtattcttctggtcggtggaggtacatggctgcagcgtcaccattgagaggatctatggggttaggataggccaataactgaggcaggaaggactcaaatatattggtaagatctatagatggagatttgaaagggtatttatcaggtaggtccactctaactttccatactccgccttcatatggtgttccttgtggtccataaaacttcactacaaattcattaagtcctcccaggatcgtaacctcatgtttactctcgatgagcttgaccacgtccgtgtccatccgcctcttgcccggactgggagatgacatggtgtcgccgccgcctctctcccttcctcggcccgtctgtcacgggcccggggccccggctctgaggagcccgcggccgcgccggctcctcggtggaggtggcaacacccccgcggtcccggcggtcccgtcagccgccgccgccgccccccgcacgggggaacaccgggcactgtccggccgggtgggggtggggaccctgcggcgcccggctcgggctgcccctctccggctgtggttccgccgcggccctgccccggcgctcctctgcgccgcgcgacgctccctcctgcctgctgtggctcgctcgcctgctccccactcaccctctgaccggctcctagcagcctccactataagcggacgactcctgctcagtcggcctccctaccccagcctcgctct

SEQ ID NO: 10752 - RNA, 26 nt, Homo sapiens
  source 1..26: mol_type = other RNA
ctcccacttccagatctttcttctgc

SEQ ID NO: 10753 - RNA, 27 nt, Homo sapiens
  source 1..27: mol_type = other RNA
ctcccacttccagatctttcttctgca

SEQ ID NO: 10754 - RNA, 311 nt, Homo sapiens
  source 1..311: mol_type = other RNA
ctccccggcctctgcccccagacagctctctcctgccaggccaccctcagtcacccaaggcccagtccaaactagaggcagaaccacccaagttggagtcccacacccacctcccagggcccaccccttccctcccaggcccttgaggcagcaatgctgagtggcttgagggcctcaggctcccggcctggcagggttgtcaccctctggccagccctggaggggacggcgcagcaagaggcagcgaggacagcttggattctcctgggtttgggcactcacccccggggctgtggaggcaggagcgtcct

SEQ ID NO: 10755 - RNA, 1277 nt, Homo sapiens
  source 1..1277: mol_type = other RNA
ctccccggcctctgcccccagaggggatggaagcgtcctggtcctccccttccgtgtggtcctggaattgcgggctgctctgagcctcacttcctgtggccactcctgcctctcccaaagcctgggcctgcagggggctgtcgccaacctcggtgggcgcggagaggccgtcaccctccagtggcgtggtggctgtgcctgggggctggctcggctggccagtggggccactctgctgggcttggctgtggggcagggctgtgtcctgaggccacgggtttgaaagcaaagtcaggtgacaggggctggcaggagaaaggggcaaggaagccagctctgaggaagcggacttgttccccttctttttcttcttccttttcttctttttgctctgctcacagtctgcagaaggcacgctggcggcctcaagcggggctgcatcctgcttccttctcttgctgggtatggcattagcagcttcccattcatcggatatgaggtctacagcagcatctaccaaaacctctgatgtagctccttcttggacggtccaggaggctttggaacagggctcctcggggttttcttgccaactgtctgagcccgggaacaagcacgggcccccttcctccttcagctcctgcccacactccatttcaccctccgaggccgacgccattgtggagttattgttctcagaatctgctatgggggctgcaggaggcagcctctctccgcactggctgcagaacttgggggtttcctccttggagacatgctggcacgaaggacactccatgggtcctgctgggactgccctgcagatccagaagcaagagcaggagtcgctggcagcctgctatatactacatgtcctgtcacgtgaccacggcttcagtttcattttcctggccttgagccccgcgctcgggcgacttcgccaagtcggaaggacgctgcgcggtgcggttcagacggggcgatgcctccctcgtaaaagttaggagtctgtttttgcaacttcacttttccgttgttgccattcgtacaggcgcaggattcccgggcggacctgcaggcccgggtccggctgtccccttccactacaccccccgtgccccggccacttcccgggggcagcactgccggggcgcaaagcctcctccgcgctctgcgctccggggatgtcgccggggtcccaggcgtgcccgctgcccccaccccgacccctcccgcagccggggaacagggtcagtgggcgccgcgggcggggctgg

SEQ ID NO: 10756 - RNA, 990 nt, Homo sapiens
  source 1..990: mol_type = other RNA
ctccccggcctctgcccccagaggggatggaagcgtcctggtcctccccttccgtgtggtcctggaattgcgggctgctctgagcctcacttcctgtggccactcctgcctctcccaaagcctgggcctgcagggggctgtcgccaacctcggtgggcgcggagaggccgtcaccctccagtggcgtggtggctgtgcctgggggctggctcggctggccagtggggccactctgctgggcttggctgtggggcagggctgtgtcctgaggccacgggtttgaaagcaaagtcaggtgacaggggctggcaggagaaaggggcaaggaagccagctctgaggaagcggacttgttccccttctttttcttcttccttttcttctttttgctctgctcacagtctgcagaaggcacgctggcggcctcaagcggggctgcatcctgcttccttctcttgctgggtatggcattagcagcttcccattcatcggatatgaggtctacagcagcatctaccaaaacctctgatgtagctccttcttggacggtccaggaggctttggaacagggctcctcggggttttcttgccaactgtctgagcccgggaacaagcacgggcccccttcctccttcagctcctgcccacactccatttcaccctccgaggccgacgccattgtggagttattgttctcagaatctgctatgggggctgcaggaggcagcctctctccgcactggctgcagaacttgggggtttcctccttggagacatgctggcacgaaggacactccatgggtcctgctgggactgccctgcagatccagaagcaagagcaggagtcgctggcagcctgctatatactacatgtcctgtcacgtgaccacggcttcagtttcattttctgcggcccccgagctcgccgcctgccgcgcgctgtcgcccctcgggtcacggggccctgggccccgccctgcccgccgccgc

SEQ ID NO: 10757 - RNA, 894 nt, Homo sapiens
  source 1..894: mol_type = other RNA
ctccccggcctctgcccccagaggggatggaagcgtcctggtcctccccttccgtgtggtcctggaattgcgggctgctctgagcctcacttcctgtggccactcctgcctctcccaaagcctgggcctgcagggggctgtcgccaacctcggtgggcgcggagaggccgtcaccctccagtggcgtggtggctgtgcctgggggctggctcggctggccagtggggccactctgctgggcttggctgtggggcagggctgtgtcctgaggccacgggtttgaaagcaaagtcaggtgacaggggctggcaggagaaaggggcaaggaagccagctctgaggaagcggacttgttccccttctttttcttcttccttttcttctttttgctctgctcacagtctgcagaaggcacgctggcggcctcaagcggggctgcatcctgcttccttctcttgctgggtatggcattagcagcttcccattcatcggatatgaggtctacagcagcatctaccaaaacctctgatgtagctccttcttggacggtccaggaggctttggaacagggctcctcggggttttcttgccaactgtctgagcccgggaacaagcacgggcccccttcctccttcagctcctgcccacactccatttcaccctccgaggccgacgccattgtggagttattgttctcagaatctgctatgggggctgcaggaggcagcctctctccgcactggctgcagaacttgggggtttcctccttggagacatgctggcacgaaggacactccatgggtcctgctgggactgccctgcggcccccgagctcgccgcctgccgcgcgctgtcgcccctcgggtcacggggccctgggccccgccctgcccg

SEQ ID NO: 10758 - RNA, 811 nt, Homo sapiens
  source 1..811: mol_type = other RNA
ctccccggcctctgcccccagaggggatggaagcgtcctggtcctccccttccgtgtggtcctggaattgcgggctgctctgagcctcacttcctgtggccactcctgcctctcccaaagcctgggcctgcagggggctgtcgccaacctcggtgggcgcggagaggccgtcaccctccagtggcgtggtggctgtgcctgggggctggctcggctggccagtggggccactctgctgggcttggctgtggggcagggctgtgtcctgaggccacgggtttgaaagcaaagtcaggtgacaggggctggcaggagaaaggggcaaggaagccagctctgaggaagcggacttgttccccttctttttcttcttccttttcttctttttgctttcttggacggtccaggaggctttggaacagggctcctcggggttttcttgccaactgtctgagcccgggaacaagcacgggcccccttcctccttcagctcctgcccacactccatttcaccctccgaggccgacgccattgtggagttattgttctcagaatctgctatgggggctgcaggaggcagcctctctccgcactggctgcagaacttgggggtttcctccttggagacatgctggcacgaaggacactccatgggtcctgctgggactgccctgcagatccagaagcaagagcaggagtcgctggcagcctgctatatactacatgtcctgtcacgtgaccacggcttcagtttcattttctgcggcccccgagctcgccgcctgccgcgcgctgtcgcccctcgggtcac

SEQ ID NO: 10759 - RNA, 216 nt, Homo sapiens
  source 1..216: mol_type = other RNA
ctccccggcctctgcccccagcaccaggcaggcaggcaggaagaaagggcaggcttcaggcccactgccaaccctggggccagctattctgagcctggacagagcatctgatacgcccaagggcccagaaagggcacacacatgtctccgtccccctggggtccctgttttgacacccttgggcctctggggcccccccatagcttggccaggggc

SEQ ID NO: 10760 - RNA, 3390 nt, Homo sapiens
  source 1..3390: mol_type = other RNA
ctccccggcctctgcccccagcctgcagagggagaccgggaggtcagaggagcaggccgaggagaggcctgccccagggatccagcctatcctctctgagagtcaggagccaggtcctcctttgcttccaggctccctgccctgagccagcgggccgcatggagtccgtggggaggctgccaccctgccttcactctgaggttgggccgaacagcagatggcagcacacctggcaacgctgagttctagggctggtactcagacccctgtgccttcttcctgggtccactggactgtgccagagccatggcagccaataagcaccatctccaggctgtgggggtcccagggcaaggccaggccccctgaccctggtgggggctctccagtgctggtagcctcagcctggctcacaggctctgcgggcccagtcctagccccttcctcagaaggaggaggggaggcaggggtgctgggctcagagcagaggtctcctgaggcagggggctctgagtctgaggtggaggtccagaaagctgtggctcgaggccagggggagctctgagacgctgggggaccccagggccagggtgccatgaggggaggaggccccggacgagggtggggccaagtcccactcaagacagagccagctgggggctgcaggcagtaggaggatgccccagtgtccacacacagaggctgcagaagcccggaggtgctggctgggcacggcccctctcccgatgcccgagggcacggaccctccctgtggggcgccaggacaagctgcacagcctggcgaagtgactgcagtccttcccgcatctgcagcacctgctctgacagctctgtcaccgcctgccgaagcttgtccagtgtgtctgtgttccttgcctcgctgggcccatggggaacagtgagcaggccgctctctggtccaggggaggggctgctgctacattccgggccagactggcccacgcggaaagagaacttgggctggtccgagccacagccgtcttcaatgccatctactaccctggggctcagatctgggggcacattccatggcatggggggcagccgtagcccctctagggcccgtgggggagcagaggggccagcctcagccttcaaagcccctgccctgcctggcctccctctgccacctagacgaggccggggtgctgttcgacgtggggatagcagcttggcagctgaggatgaggaggtgcagccaggggacagcagggggctggagggctcatcagctggggctggggagaccgtggggccctgctccccatctgtctccttctcctccagcgtggacataagggtattgtcgccgctcagggagctggtgtccacctctgcagagcctcccccagcacccaggttgtagctgagctcccctcggaggccacgactgaagcgcggggcaaactcggggtacagcgcaaggctgtcgtgcaggccagccagctgcagacactgcaggacgcagtacgtcagccccttcacgtcggcattggcctttaccacctgctcccgccggggcagctcacagccgatcaggtcgcccttccctaggatggcgagcacggtgccacccttgagcacctccatggagccagagcagacaaagtagagggcctgcagggcatcgccttggtggatgaggtactcgcccggcgtgcagaaggcgggccgcagggccagagacagtgcccgcaggcagccgcggctggccgcctcaaacagtggcagctgcaggacctccttgtgcaggtgcatggcgatgtctgcgcgcagctcgtcagggaggctctgcagcagctcggtggtgtcgatgccattgttcaccgcccaggtggcctggaagtactccagcatgcgctgcttgaggggcttggggatacggtggatgcggatgtagtcgcgcaggtcgcgcgtgcggctgtggtacagaaagcggcgggcgtacatgcgctggatgatggccgtcacgttcccaaacaccaccgcgtgcatcagggcgccgatgagcatggtgcagatggagaagatcttctcggtgtccgtgttggcggacacgttgccgaagcccacgctggtgaggctgctgagtgcgaagtagagggaggtgatgtaggcgctgcgcagcgacgggccgcccagcagctccagccccgtcccgttggcctcgctgctgctgctgcagttgtcactctggccggagctgttccctccagctggcctccggcccaccaggtagtagggagtctccagtcggcgggccagctcctgcagccagccaatctcaggcagctcggattcgctgctctcgatctcccgctggccaatgtaaaaccagacgcaggcgacccagtgcgcgagcagggcgaacacggccatgagcagtgtcagcaccacggcgctgtactgcgagtaccggtccagccgcggaagcaggcgcagcaggcgcagcaggcgcaccgtcttcagcagatgggccccgaagtacacgttgaccttgaaggcatgtagcaggtcaaagggcagcgctgcgatgacatccagcaggaaccaggtggtgacgtagtggaggcaaatggactttggggcaaacaccacctggcccgacttggacacgaatgtggtacggaaattcagcacaatgtcaaggatgaagaggacctccacggccaggtcacagacgctgggcgggccgcgggcggcactgggctcccgtgctgtgctcacacacacgctgtagggcacagtgacagccacatagagtgtggcgagcaggatgaagccatcccaggtggctctcagtgccccacagtgcaacaggatgaagggcgacttccggatggcggctactttgtactcaggcaagtttggtttctccccaaacacccccttattgagcttgtgcttgcccttgggctgcttctgcaggtgcccggacaggtggtagagcacggcccggctccgccgccggttggcattgaagcctttggatcgtgcccggccatatcggcgccggccaccacctcacagggccagggtggagaactagcaggaggccgtcagcagaggtgtgggaacttacagcaggagcccaggagctgtctccttccatctgtcggggccccctcggttcttggtttcgctgatgtccttgtgagagactaggaagagagccacctcccctttctcattctttatgggtatcacatccaggagacaccagaacgggagcccgctcttccggtacaggatcagctcagccttgaactccttgtgctcgtccagggccttgcggatctgttggcggacgagctcactggtgtctggcccataaaggaaggagcaggc

SEQ ID NO: 10761 - RNA, 3897 nt, Homo sapiens
  source 1..3897: mol_type = other RNA
ctccccggcctctgcccccagcctgcagagggagaccgggaggtcagaggagcaggccgaggagaggcctgccccagggatccagcctatcctctctgagagtcaggagccaggtcctcctttgcttccaggctccctgccctgagccagcgggccgcatggagtccgtggggaggctgccaccctgccttcactctgaggttgggccgaacagcagatggcagcacacctggcaacgctgagttctagggctggtactcagacccctgtgccttcttcctgggtccactggactgtgccagagccatggcagccaataagcaccatctccaggctgtgggggtcccagggcaaggccaggccccctgaccctggtgggggctctccagtgctggtagcctcagcctggctcacaggctctgcgggcccagtcctagccccttcctcagaaggaggaggggaggcaggggtgctgggctcagagcagaggtctcctgaggcagggggctctgagtctgaggtggaggtccagaaagctgtggctcgaggccagggggagctctgagacgctgggggaccccagggccagggtgccatgaggggaggaggccccggacgagggtggggccaagtcccactcaagacagagccagctgggggctgcaggcagtaggaggatgccccagtgtccacacacagaggctgcagaagcccggaggtgctggctgggcacggcccctctcccgatgcccgagggcacggaccctccctgtggggcgccaggacaagctgcacagcctggcgaagtgactgcagtccttcccgcatctgcagcacctgctctgacagctctgtcaccgcctgccgaagcttgtccagtgtgtctgtgttccttgcctcgctgggcccatggggaacagtgagcaggccgctctctggtccaggggaggggctgctgctacattccgggccagactggcccacgcggaaagagaacttgggctggtccgagccacagccgtcttcaatgccatctactaccctggggctcagatctgggggcacattccatggcatggggggcagccgtagcccctctagggcccgtgggggagcagaggggccagcctcagccttcaaagcccctgccctgcctggcctccctctgccacctagacgaggccggggtgctgttcgacgtggggatagcagcttggcagctgaggatgaggaggtgcagccaggggacagcagggggctggagggctcatcagctggggctggggagaccgtggggccctgctccccatctgtctccttctcctccagcgtggacataagggtattgtcgccgctcagggagctggtgtccacctctgcagagcctcccccagcacccaggttgtagctgagctcccctcggaggccacgactgaagcgcggggcaaactcggggtacagcgcaaggctgtcgtgcaggccagccagctgcagacactgcaggacgcagtacgtcagccccttcacgtcggcattggcctttaccacctgctcccgccggggcagctcacagccgatcaggtcgcccttccctaggatggcgagcacggtgccacccttgagcacctccatggagccagagcagacaaagtagagggcctgcagggcatcgccttggtggatgaggtactcgcccggcgtgcagaaggcgggccgcagggccagagacagtgcccgcaggcagccgcggctggccgcctcaaacagtggcagctgcaggacctccttgtgcaggtgcatggcgatgtctgcgcgcagctcgtcagggaggctctgcagcagctcggtggtgtcgatgccattgttcaccgcccaggtggcctggaagtactccagcatgcgctgcttgaggggcttggggatacggtggatgcggatgtagtcgcgcaggtcgcgcgtgcggctgtggtacagaaagcggcgggcgtacatgcgctggatgatggccgtcacgttcccaaacaccaccgcgtgcatcagggcgccgatgagcatggtgcagatggagaagatcttctcggtgtccgtgttggcggacacgttgccgaagcccacgctggtgaggctgctgagtgcgaagtagagggaggtgatgtaggcgctgcgcagcgacgggccgcccagcagctccagccccgtcccgttggcctcgctgctgctgctgcagttgtcactctggccggagctgttccctccagctggcctccggcccaccaggtagtagggagtctccagtcggcgggccagctcctgcagccagccaatctcaggcagctcggattcgctgctctcgatctcccgctggccaatgtaaaaccagacgcaggcgacccagtgcgcgagcagggcgaacacggccatgagcagtgtcagcaccacggcgctgtactgcgagtaccggtccagccgcggaagcaggcgcagcaggcgcagcaggcgcaccgtcttcagcagatgggccccgaagtacacgttgaccttgaaggcatgtagcaggtcaaagggcagcgctgcgatgacatccagcaggaaccaggtggtgacgtagtggaggcaaatggactttggggcaaacaccacctggcccgacttggacacgaatgtggtacggaaattcagcacaatgtcaaggatgaagaggacctccacggccaggtcacagacgctgggcgggccgcgggcggcactgggctcccgtgctgtgctcacacacacgctgtagggcacagtgacagccacatagagtgtggcgagcaggatgaagccatcccaggtggctctcagtgccccacagtgcaacaggatgaagggcgacttccggatggcggctactttgtactcaggcaagtttggtttctccccaaacacccccttattgagcttgtgcttgcccttgggctgcttctgcaggtgcccggacaggtggtagagcacggcccggctccgccgccggttggcattgaagcctttggatcgtgcccggccatatcggcgccggccaccacctgtctccttccatctgtcggggccccctcggttcttggtttcgctgatgtccttgtgagagactaggaagagagccacctcccctttctcattctttatgggtatcacatccaggagacaccagaacgggagcccgctcttccggtacaggatcagctcagccttgaactccttgtgctcgtccagggccttgcggatctgttggcggacgagctcactggtgtctggcccataaaggaaggagcaggcacagccccgctgcatgacctcagcccgggagaagcccgtgaggtcacagaagccatcagagcagtagaccacggggaagagccccgccacctgggcgttgcccagcacgaagttactgtgcgtgccgtcgaagcgcgtagcgatggtgtccaggaaggtgttctgcggcgccaggaggccccgcatggccggcatcttaggcgcccgcggctgcccgccccatccctccggggtgcggggactccgcgccgggggagggcgcccagctcggccgccccccgccgggccccgcgctccctagcgcagccgtcggggggcaatgcgcagaccgggatccggggtcgcgccggacgctggcgcgcgagggggcgtccgcgccgtcggggcccggagcatggcgcgcggcccctcgcgccctcgccgcccacaaatcccgggctccaggccccgcggccgccgcgctctcagcacctcccgccgcggcagcggctcgcgtgtcggctgcgggtgggcttccgctcggcttcgctcggcgccggctctcggcagctccctccgtctgtcggggagaagctgcagcct

SEQ ID NO: 10762 - RNA, 3893 nt, Homo sapiens
  source 1..3893: mol_type = other RNA
ctccccggcctctgcccccagcctgcagagggagaccgggaggtcagaggagcaggccgaggagaggcctgccccagggatccagcctatcctctctgagagtcaggagccaggtcctcctttgcttccaggctccctgccctgagccagcgggccgcatggagtccgtggggaggctgccaccctgccttcactctgaggttgggccgaacagcagatggcagcacacctggcaacgctgagttctagggctggtactcagacccctgtgccttcttcctgggtccactggactgtgccagagccatggcagccaataagcaccatctccaggctgtgggggtcccagggcaaggccaggccccctgaccctggtgggggctctccagtgctggtagcctcagcctggctcacaggctctgcgggcccagtcctagccccttcctcagaaggaggaggggaggcaggggtgctgggctcagagcagaggtctcctgaggcagggggctctgagtctgaggtggaggtccagaaagctgtggctcgaggccagggggagctctgagacgctgggggaccccagggccagggtgccatgaggggaggaggccccggacgagggtggggccaagtcccactcaagacagagccagctgggggctgcaggcagtaggaggatgccccagtgtccacacacagaggctgcagaagcccggaggtgctggctgggcacggcccctctcccgatgcccgagggcacggaccctccctgtggggcgccaggacaagctgcacagcctggcgaagtgactgcagtccttcccgcatctgcagcacctgctctgacagctctgtcaccgcctgccgaagcttgtccagtgtgtctgtgttccttgcctcgctgggcccatggggaacagtgagcaggccgctctctggtccaggggaggggctgctgctacattccgggccagactggcccacgcggaaagagaacttgggctggtccgagccacagccgtcttcaatgccatctactaccctggggctcagatctgggggcacattccatggcatggggggcagccgtagcccctctagggcccgtgggggagcagaggggccagcctcagccttcaaagcccctgccctgcctggcctccctctgccacctagacgaggccggggtgctgttcgacgtggggatagcagcttggcagctgaggatgaggaggtgcagccaggggacagcagggggctggagggctcatcagctggggctggggagaccgtggggccctgctccccatctgtctccttctcctccagcgtggacataagggtattgtcgccgctcagggagctggtgtccacctctgcagagcctcccccagcacccaggttgtagctgagctcccctcggaggccacgactgaagcgcggggcaaactcggggtacagcgcaaggctgtcgtgcaggccagccagctgcagacactgcaggacgcagtacgtcagccccttcacgtcggcattggcctttaccacctgctcccgccggggcagctcacagccgatcaggtcgcccttccctaggatggcgagcacggtgccacccttgagcacctccatggagccagagcagacaaagtagagggcctgcagggcatcgccttggtggatgaggtactcgcccggcgtgcagaaggcgggccgcagggccagagacagtgcccgcaggcagccgcggctggccgcctcaaacagtggcagctgcaggacctccttgtgcaggtgcatggcgatgtctgcgcgcagctcgtcagggaggctctgcagcagctcggtggtgtcgatgccattgttcaccgcccaggtggcctggaagtactccagcatgcgctgcttgaggggcttggggatacggtggatgcggatgtagtcgcgcaggtcgcgcgtgcggctgtggtacagaaagcggcgggcgtacatgcgctggatgatggccgtcacgttcccaaacaccaccgcgtgcatcagggcgccgatgagcatggtgcagatggagaagatcttctcggtgtccgtgttggcggacacgttgccgaagcccacgctggtgaggctgctgagtgcgaagtagagggaggtgatgtaggcgctgcgcagcgacgggccgcccagcagctccagccccgtcccgttggcctcgctgctgctgctgcagttgtcactctggccggagctgttccctccagctggcctccggcccaccaggtagtagggagtctccagtcggcgggccagctcctgcagccagccaatctcaggcagctcggattcgctgctctcgatctcccgctggccaatgtaaaaccagacgcaggcgacccagtgcgcgagcagggcgaacacggccatgagcagtgtcagcaccacggcgctgtactgcgagtaccggtccagccgcggaagcaggcgcagcaggcgcagcaggcgcaccgtcttcagcagatgggccccgaagtacacgttgaccttgaaggcatgtagcaggtcaaagggcagcgctgcgatgacatccagcaggaaccaggtggtgacgtagtggaggcaaatggactttggggcaaacaccacctggcccgacttggacacgaatgtggtacggaaattcagcacaatgtcaaggatgaagaggacctccacggccaggtcacagacgctgggcgggccgcgggcggcactgggctcccgtgctgtgctcacacacacgctgtagggcacagtgacagccacatagagtgtggcgagcaggatgaagccatcccaggtggctctcagtgccccacagtgcaacaggatgaagggcgacttccggatggcggctactttgtactcaggcaagtttggtttctccccaaacacccccttattgagcttgtgcttgcccttgggctgcttctgcaggtgcccggacaggtggtagagcacggcccggctccgccgccggttggcattgaagcctttggatcgtgcccggccatatcggcgccggccaccacctgtctccttccatctgtcggggccccctcggttcttggtttcgctgatgtccttgtgagagactaggaagagagccacctcccctttctcattctttatgggtatcacatccaggagacaccagaacgggagcccgctcttccggtacaggatcagctcagccttgaactccttgtgctcgtccagggccttgcggatctgttggcggacgagctcactggtgtctggcccataaaggaaggagcaggcacagccccgctgcatgacctcagcccgggagaagcccgtgaggtcacagaagccatcagagcagtagaccacggggaagagccccgccacctgggcgttgcccagcacgaagttagcgtgccgtcgaagcgcgtagcgatggtgtccaggaaggtgttctgcggcgccaggaggccccgcatggccggcatcttaggcgcccgcggctgcccgccccatccctccggggtgcggggactccgcgccgggggagggcgcccagctcggccgccccccgccgggccccgcgctccctagcgcagccgtcggggggcaatgcgcagaccgggatccggggtcgcgccggacgctggcgcgcgagggggcgtccgcgccgtcggggcccggagcatggcgcgcggcccctcgcgccctcgccgcccacaaatcccgggctccaggccccgcggccgccgcgctctcagcacctcccgccgcggcagcggctcgcgtgtcggctgcgggtgggcttccgctcggcttcgctcggcgccggctctcggcagctccctccgtctgtcggggagaagctgcagcct

SEQ ID NO: 10763 - RNA, 4554 nt, Homo sapiens
  source 1..4554: mol_type = other RNA
ctccccggcctctgcccccagcctgcagagggagaccgggaggtcagaggagcaggccgaggagaggcctgccccagggatccagcctatcctctctgagagtcaggagccaggtcctcctttgcttccaggctccctgccctgagccagcgggccgcatggagtccgtggggaggctgccaccctgccttcactctgaggttgggccgaacagcagatggcagcacacctggcaacgctgagttctagggctggtactcagacccctgtgccttcttcctgggtccactggactgtgccagagccatggcagccaataagcaccatctccaggctgtgggggtcccagggcaaggccaggccccctgaccctggtgggggctctccagtgctggtagcctcagcctggctcacaggctctgcgggcccagtcctagccccttcctcagaaggaggaggggaggcaggggtgctgggctcagagcagaggtctcctgaggcagggggctctgagtctgaggtggaggtccagaaagctgtggctcgaggccagggggagctctgagacgctgggggaccccagggccagggtgccatgaggggaggaggccccggacgagggtggggccaagtcccactcaagacagagccagctgggggctgcaggcagtaggaggatgccccagtgtccacacacagaggctgcagaagcccggaggtgctggctgggcacggcccctctcccgatgcccgagggcacggaccctccctgtggggcgccaggacaagctgcacagcctggcgaagtgactgcagtccttcccgcatctgcagcacctgctctgacagctctgtcaccgcctgccgaagcttgtccagtgtgtctgtgttccttgcctcgctgggcccatggggaacagtgagcaggccgctctctggtccaggggaggggctgctgctacattccgggccagactggcccacgcggaaagagaacttgggctggtccgagccacagccgtcttcaatgccatctactaccctgtgaacccaggtaccaggacaacaaatcaatggacaggcagccactgtggggtcatacgggacgggatgccccagcgtccacacacacaggctgcaggagcgtggaactgaccaggagcccaggagaaagctaacatggggtcccttcccctaggagcttacagtttagctggggggccaagcttgagcagcatgagatgcaagagttcagagcagcgtgtgccacacaccacacagtggagtgggacagcaggagaaaggaggagcacagaaggcttcctggaggaggcaggcttggcccacatagactagcgggagttaagatggttagatgggcacctagggcagggtgcgcctgcccagggcctcagcctcatcaccaccatctctgccacgggggcctagggtctgctcacctggggctcagatctgggggcacattccatggcatggggggcagccgtagcccctctagggcccgtgggggagcagaggggccagcctcagccttcaaagcccctgccctgcctggcctccctctgccacctagacgaggccggggtgctgttcgacgtggggatagcagcttggcagctgaggatgaggaggtgcagccaggggacagcagggggctggagggctcatcagctggggctggggagaccgtggggccctgctccccatctgtctccttctcctccagcgtggacataagggtattgtcgccgctcagggagctggtgtccacctctgcagagcctcccccagcacccaggttgtagctgagctcccctcggaggccacgactgaagcgcggggcaaactcggggtacagcgcaaggctgtcgtgcaggccagccagctgcagacactgcaggacgcagtacgtcagccccttcacgtcggcattggcctttaccacctgctcccgccggggcagctcacagccgatcaggtcgcccttccctcggtggtgtcgatgccattgttcaccgcccaggtggcctggaagtactccagcatgcgctgcttgaggggcttggggatacggtggatgcggatgtagtcgcgcaggtcgcgcgtgcggctgtggtacagaaagcggcgggcgtacatgcgctggatgatggccgtcacgttcccaaacaccaccgcgtgcatcagggcgccgatgagcatggtgcagatggagaagatcttctcggtgtccgtgttggcggacacgttgccgaagcccacgctggtgaggctgctgagtgcgaagtagagggaggtgatgtaggcgctgcgcagcgacgggccgcccagcagctccagccccgtcccgttggcctcgctgctgctgctgcagttgtcactctggccggagctgttccctccagctggcctccggcccaccaggtagtagggagtctccagtcggcgggccagctcctgcagccagccaatctcaggcagctcggattcgctgctctcgatctcccgctggccaatgtaaaaccagacgcaggcgacccagtgcgcgagcagggcgaacacggccatgagcagtgtcagcaccacggcgctgtactgcgagtaccggtccagccgcggaagcaggcgcagcaggcgcagcaggcgcaccgtcttcagcagatgggccccgaagtacacgttgaccttgaaggcatgtagcaggtcaaagggcagcgctgcgatgacatccagcaggaaccaggtggtgacgtagtggaggcaaatggactttggggcaaacaccacctggcccgacttggacacgaatgtggtacggaaattcagcacaatgtcaaggatgaagaggacctccacggccaggtcacagacgctgggcgggccgcgggcggcactgggctcccgtgctgtgctcacacacacgctgtagggcacagtgacagccacatagagtgtggcgagcaggatgaagccatcccaggtggctctcagtgccccacagtgcaacaggatgaagggcgacttccggatggcggctactttgtactcaggcaagtttggtttctccccaaacacccccttattgagcttgtgcttgcccttgggctgcttctgcaggtgcccggacaggtggtagagcacggcccggctccgccgccggttggcattgaagcctttggatcgtgcccggccatatcggcgccggccaccacctgtctccttccatctgtcggggccccctcggttcttggtttcgctgatgtccttgtgagagactaggaagagagccacctcccctttctcattctttatgggtatcacatccaggagacaccagaacgggagcccgctcttccggtacaggatcagctcagccttgaactccttgtgctcgtccagggccttgcggatctgttggcggacgagctcactggtgtctggcccataaaggaaggagcaggcacagccccgctgcatgacctcagcccgggagaagcccgtgaggtcacagaagccatcagagcagtagaccacggggaagagccccgccacctgggcgttgcccagcacgaagttactgtgcgtgccgtcgaagcgcgtagcgatggtgtccaggaaggtgttctgcggcgccaggaggccccgcatggccggcatcttaggcgcccgcggctgcccgccccatccctccggggtgcggggactccgcgccgggggagggcgcccagctcggccgccccccgccgggccccgcgctccctagcgcagccgtcggggggcaatgcgcagaccgggatccggggtcgcgccggacgctggcgcgcgagggggcgtccgcgccgtcggggcccggagcatggcgcgcggcccctcgcgccctcgccgcccacaaatcccgggctccaggccccgcggccgccgcgctctcagcacctcccgccgcggcagcggctcgcgtgtcggctgcgggtgggcttccgctcggcttcgctcggcgccggctctcggcagctccctccgtctgtcggggagaagctgcagcctccctccctccctcccgcgcccgccgcctgcaccggggtaaccatggagacggggcacacccagccagggccgcctccttaaagggacaggcctcccgcggagggctcccctcccttcgggacctcggcgggggcggggaggtggcggccgccctgatcccaccccgcgggcctccccgcccgtacctcggagaaccactggcgagcggccggccccctttggctcactcggcctcagccgcagaggggaggcgtctttctctgcagcccgggggctctccgagagcctcctagcagcctctcctcccccggcggaatgggaggggggctcggggcgtggggggcaggggacgcatgctgtggaagatgctctccccgaggaaaatgcagtgggcaaggggacagggcgacaggcgcaggtgaaggccctgcggccagcggaggccggcgctctagaggggctccagccgcacccgggaaatctaaaagc

SEQ ID NO: 10764 - RNA, 4419 nt, Homo sapiens
  source 1..4419: mol_type = other RNA
ctccccggcctctgcccccagcctgcagagggagaccgggaggtcagaggagcaggccgaggagaggcctgccccagggatccagcctatcctctctgagagtcaggagccaggtcctcctttgcttccaggctccctgccctgagccagcgggccgcatggagtccgtggggaggctgccaccctgccttcactctgaggttgggccgaacagcagatggcagcacacctggcaacgctgagttctagggctggtactcagacccctgtgccttcttcctgggtccactggactgtgccagagccatggcagccaataagcaccatctccaggctgtgggggtcccagggcaaggccaggccccctgaccctggtgggggctctccagtgctggtagcctcagcctggctcacaggctctgcgggcccagtcctagccccttcctcagaaggaggaggggaggcaggggtgctgggctcagagcagaggtctcctgaggcagggggctctgagtctgaggtggaggtccagaaagctgtggctcgaggccagggggagctctgagacgctgggggaccccagggccagggtgccatgaggggaggaggccccggacgagggtggggccaagtcccactcaagacagagccagctgggggctgcaggcagtaggaggatgccccagtgtccacacacagaggctgcagaagcccggaggtgctggctgggcacggcccctctcccgatgcccgagggcacggaccctccctgtggggcgccaggacaagctgcacagcctggcgaagtgactgcagtccttcccgcatctgcagcacctgctctgacagctctgtcaccgcctgccgaagcttgtccagtgtgtctgtgttccttgcctcgctgggcccatggggaacagtgagcaggccgctctctgtgggtagtaggatggggttatcagctggggctggtccaggggaggggctgctgctacattccgggccagactggcccacgcggaaagagaacttgggctggtccgagccacagccgtcttcaatgccatctactaccctggggctcagatctgggggcacattccatggcatggggggcagccgtagcccctctagggcccgtgggggagcagaggggccagcctcagccttcaaagcccctgccctgcctggcctccctctgccacctagacgaggccggggtgctgttcgacgtggggatagcagcttggcagctgaggatgaggaggtgcagccaggggacagcagggggctggagggctcatcagctggggctggggagaccgtggggccctgctccccatctgtctccttctcctccagcgtggacataagggtattgtcgccgctcagggagctggtgtccacctctgcagagcctcccccagcacccaggttgtagctgagctcccctcggaggccacgactgaagcgcggggcaaactcggggtacagcgcaaggctgtcgtgcaggccagccagctgcagacactgcaggacgcagtacgtcagccccttcacgtcggcattggcctttaccacctgctcccgccggggcagctcacagccgatcaggtcgcccttccctaggatggcgagcacggtgccacccttgagcacctccatggagccagagcagacaaagtagagggcctgcagggcatcgccttggtggatgaggtactcgcccggcgtgcagaaggcgggccgcagggccagagacagtgcccgcaggcagccgcggctggccgcctcaaacagtggcagctgcaggacctccttgtgcaggtgcatggcgatgtctgcgcgcagctcgtcagggaggctctgcagcagctcggtggtgtcgatgccattgttcaccgcccaggtggcctggaagtactccagcatgcgctgcttgaggggcttggggatacggtggatgcggatgtagtcgcgcaggtcgcgcgtgcggctgtggtacagaaagcggcgggcgtacatgcgctggatgatggccgtcacgttcccaaacaccaccgcgtgcatcagggcgccgatgagcatggtgcagatggagaagatcttctcggtgtccgtgttggcggacacgttgccgaagcccacgctggtgaggctgctgagtgcgaagtagagggaggtgatgtaggcgctgcgcagcgacgggccgcccagcagctccagccccgtcccgttggcctcgctgctgctgctgcagttgtcactctggccggagctgttccctccagctggcctccggcccaccaggtagtagggagtctccagtcggcgggccagctcctgcagccagccaatctcaggcagctcggattcgctgctctcgatctcccgctggccaatgtaaaaccagacgcaggcgacccagtgcgcgagcagggcgaacacggccatgagcagtgtcagcaccacggcgctgtactgcgagtaccggtccagccgcggaagcaggcgcagcaggcgcagcaggcgcaccgtcttcagcagatgggccccgaagtacacgttgaccttgaaggcatgtagcaggtcaaagggcagcgctgcgatgacatccagcaggaaccaggtggtgacgtagtggaggcaaatggactttggggcaaacaccacctggcccgacttggacacgaatgtggtacggaaattcagcacaatgtcaaggatgaagaggacctccacggccaggtcacagacgctgggcgggccgcgggcggcactgggctcccgtgctgtgctcacacacacgctgtagggcacagtgacagccacatagagtgtggcgagcaggatgaagccatcccaggtggctctcagtgccccacagtgcaacaggatgaagggcgacttccggatggcggctactttgtactcaggcaagtttggtttctccccaaacacccccttattgagcttgtgcttgcccttgggctgcttctgcaggtgcccggacaggtggtagagcacggcccggctccgccgccggttggcattgaagcctttggatcgtgcccggccatatcggcgccggccaccacctgtctccttccatctgtcggggccccctcggttcttggtttcgctgatgtccttgtgagagactaggaagagagccacctcccctttctcattctttatgggtatcacatccaggagacaccagaacgggagcccgctcttccggtacaggatcagctcagccttgaactccttgtgctcgtccagggccttgcggatctgttggcggacgagctcactggtgtctggcccataaaggaaggagcaggcacagccccgctgcatgacctcagcccgggagaagcccgtgaggtcacagaagccatcagagcagtagaccacggggaagagccccgccacctgggcgttgcccagcacgaagttactgtgcgtgccgtcgaagcgcgtagcgatggtgtccaggaaggtgttctgcggcgccaggaggccccgcatggccggcatcttaggcgcccgcggctgcccgccccatccctccggggtgcggggactccgcgccgggggagggcgcccagctcggccgccccccgccgggccccgcgctccctagcgcagccgtcggggggcaatgcgcagaccgggatccggggtcgcgccggacgctggcgcgcgagggggcgtccgcgccgtcggggcccggagcatggcgcgcggcccctcgcgccctcgccgcccacaaatcccgggctccaggccccgcggccgccgcgctctcagcacctcccgccgcggcagcggctcgcgtgtcggctgcgggtgggcttccgctcggcttcgctcggcgccggctctcggcagctccctccgtctgtcggggagaagctgcagcctccctccctccctcccgcgcccgccgcctgcaccggggtaaccatggagacggggcacacccagccagggccgcctccttaaagggacaggcctcccgcggagggctcccctcccttcgggacctcggcgggggcggggaggtggcggccgccctgatcccaccccgcgggcctccccgcccgtacctcggagaaccactggcgagcggccggccccctttggctcactcggcctcagccgcagaggggaggcgtctttctctgcagcccgggggctctccgagagcctcctagcagcctctcctcccccggcggaatgggaggggggctcggggcgtggggggcaggggacgcatgctgtggaagatgctctccccgaggaaaatgcagtgggcaaggggacagggcgacaggcgcaggtgaaggccctgcggccagcggaggccggcgctctagaggggctccagccgcacccgggaaatctaaaagc

SEQ ID NO: 10765 - RNA, 4415 nt, Homo sapiens
  source 1..4415: mol_type = other RNA
ctccccggcctctgcccccagcctgcagagggagaccgggaggtcagaggagcaggccgaggagaggcctgccccagggatccagcctatcctctctgagagtcaggagccaggtcctcctttgcttccaggctccctgccctgagccagcgggccgcatggagtccgtggggaggctgccaccctgccttcactctgaggttgggccgaacagcagatggcagcacacctggcaacgctgagttctagggctggtactcagacccctgtgccttcttcctgggtccactggactgtgccagagccatggcagccaataagcaccatctccaggctgtgggggtcccagggcaaggccaggccccctgaccctggtgggggctctccagtgctggtagcctcagcctggctcacaggctctgcgggcccagtcctagccccttcctcagaaggaggaggggaggcaggggtgctgggctcagagcagaggtctcctgaggcagggggctctgagtctgaggtggaggtccagaaagctgtggctcgaggccagggggagctctgagacgctgggggaccccagggccagggtgccatgaggggaggaggccccggacgagggtggggccaagtcccactcaagacagagccagctgggggctgcaggcagtaggaggatgccccagtgtccacacacagaggctgcagaagcccggaggtgctggctgggcacggcccctctcccgatgcccgagggcacggaccctccctgtggggcgccaggacaagctgcacagcctggcgaagtgactgcagtccttcccgcatctgcagcacctgctctgacagctctgtcaccgcctgccgaagcttgtccagtgtgtctgtgttccttgcctcgctgggcccatggggaacagtgagcaggccgctctctgtgggtagtaggatggggttatcagctggggctggtccaggggaggggctgctgctacattccgggccagactggcccacgcggaaagagaacttgggctggtccgagccacagccgtcttcaatgccatctactaccctggggctcagatctgggggcacattccatggcatggggggcagccgtagcccctctagggcccgtgggggagcagaggggccagcctcagccttcaaagcccctgccctgcctggcctccctctgccacctagacgaggccggggtgctgttcgacgtggggatagcagcttggcagctgaggatgaggaggtgcagccaggggacagcagggggctggagggctcatcagctggggctggggagaccgtggggccctgctccccatctgtctccttctcctccagcgtggacataagggtattgtcgccgctcagggagctggtgtccacctctgcagagcctcccccagcacccaggttgtagctgagctcccctcggaggccacgactgaagcgcggggcaaactcggggtacagcgcaaggctgtcgtgcaggccagccagctgcagacactgcaggacgcagtacgtcagccccttcacgtcggcattggcctttaccacctgctcccgccggggcagctcacagccgatcaggtcgcccttccctaggatggcgagcacggtgccacccttgagcacctccatggagccagagcagacaaagtagagggcctgcagggcatcgccttggtggatgaggtactcgcccggcgtgcagaaggcgggccgcagggccagagacagtgcccgcaggcagccgcggctggccgcctcaaacagtggcagctgcaggacctccttgtgcaggtgcatggcgatgtctgcgcgcagctcgtcagggaggctctgcagcagctcggtggtgtcgatgccattgttcaccgcccaggtggcctggaagtactccagcatgcgctgcttgaggggcttggggatacggtggatgcggatgtagtcgcgcaggtcgcgcgtgcggctgtggtacagaaagcggcgggcgtacatgcgctggatgatggccgtcacgttcccaaacaccaccgcgtgcatcagggcgccgatgagcatggtgcagatggagaagatcttctcggtgtccgtgttggcggacacgttgccgaagcccacgctggtgaggctgctgagtgcgaagtagagggaggtgatgtaggcgctgcgcagcgacgggccgcccagcagctccagccccgtcccgttggcctcgctgctgctgctgcagttgtcactctggccggagctgttccctccagctggcctccggcccaccaggtagtagggagtctccagtcggcgggccagctcctgcagccagccaatctcaggcagctcggattcgctgctctcgatctcccgctggccaatgtaaaaccagacgcaggcgacccagtgcgcgagcagggcgaacacggccatgagcagtgtcagcaccacggcgctgtactgcgagtaccggtccagccgcggaagcaggcgcagcaggcgcagcaggcgcaccgtcttcagcagatgggccccgaagtacacgttgaccttgaaggcatgtagcaggtcaaagggcagcgctgcgatgacatccagcaggaaccaggtggtgacgtagtggaggcaaatggactttggggcaaacaccacctggcccgacttggacacgaatgtggtacggaaattcagcacaatgtcaaggatgaagaggacctccacggccaggtcacagacgctgggcgggccgcgggcggcactgggctcccgtgctgtgctcacacacacgctgtagggcacagtgacagccacatagagtgtggcgagcaggatgaagccatcccaggtggctctcagtgccccacagtgcaacaggatgaagggcgacttccggatggcggctactttgtactcaggcaagtttggtttctccccaaacacccccttattgagcttgtgcttgcccttgggctgcttctgcaggtgcccggacaggtggtagagcacggcccggctccgccgccggttggcattgaagcctttggatcgtgcccggccatatcggcgccggccaccacctgtctccttccatctgtcggggccccctcggttcttggtttcgctgatgtccttgtgagagactaggaagagagccacctcccctttctcattctttatgggtatcacatccaggagacaccagaacgggagcccgctcttccggtacaggatcagctcagccttgaactccttgtgctcgtccagggccttgcggatctgttggcggacgagctcactggtgtctggcccataaaggaaggagcaggcacagccccgctgcatgacctcagcccgggagaagcccgtgaggtcacagaagccatcagagcagtagaccacggggaagagccccgccacctgggcgttgcccagcacgaagttagcgtgccgtcgaagcgcgtagcgatggtgtccaggaaggtgttctgcggcgccaggaggccccgcatggccggcatcttaggcgcccgcggctgcccgccccatccctccggggtgcggggactccgcgccgggggagggcgcccagctcggccgccccccgccgggccccgcgctccctagcgcagccgtcggggggcaatgcgcagaccgggatccggggtcgcgccggacgctggcgcgcgagggggcgtccgcgccgtcggggcccggagcatggcgcgcggcccctcgcgccctcgccgcccacaaatcccgggctccaggccccgcggccgccgcgctctcagcacctcccgccgcggcagcggctcgcgtgtcggctgcgggtgggcttccgctcggcttcgctcggcgccggctctcggcagctccctccgtctgtcggggagaagctgcagcctccctccctccctcccgcgcccgccgcctgcaccggggtaaccatggagacggggcacacccagccagggccgcctccttaaagggacaggcctcccgcggagggctcccctcccttcgggacctcggcgggggcggggaggtggcggccgccctgatcccaccccgcgggcctccccgcccgtacctcggagaaccactggcgagcggccggccccctttggctcactcggcctcagccgcagaggggaggcgtctttctctgcagcccgggggctctccgagagcctcctagcagcctctcctcccccggcggaatgggaggggggctcggggcgtggggggcaggggacgcatgctgtggaagatgctctccccgaggaaaatgcagtgggcaaggggacagggcgacaggcgcaggtgaaggccctgcggccagcggaggccggcgctctagaggggctccagccgcacccgggaaatctaaaagc

SEQ ID NO: 10766 - RNA, 4185 nt, Homo sapiens
  source 1..4185: mol_type = other RNA
ctccccggcctctgcccccagcctgcagagggagaccgggaggtcagaggagcaggccgaggagaggcctgccccagggatccagcctatcctctctgagagtcaggagccaggtcctcctttgcttccaggctccctgccctgagccagcgggccgcatggagtccgtggggaggctgccaccctgccttcactctgaggttgggccgaacagcagatggcagcacacctggcaacgctgagttctagggctggtactcagacccctgtgccttcttcctgggtccactggactgtgccagagccatggcagccaataagcaccatctccaggctgtgggggtcccagggcaaggccaggccccctgaccctggtgggggctctccagtgctggtagcctcagcctggctcacaggctctgcgggcccagtcctagccccttcctcagaaggaggaggggaggcaggggtgctgggctcagagcagaggtctcctgaggcagggggctctgagtctgaggtggaggtccagaaagctgtggctcgaggccagggggagctctgagacgctgggggaccccagggccagggtgccatgaggggaggaggccccggacgagggtggggccaagtcccactcaagacagagccagctgggggctgcaggcagtaggaggatgccccagtgtccacacacagaggctgcagaagcccggaggtgctggctgggcacggcccctctcccgatgcccgagggcacggaccctccctgtggggcgccaggacaagctgcacagcctggcgaagtgactgcagtccttcccgcatctgcagcacctgctctgacagctctgtcaccgcctgccgaagcttgtccagtgtgtctgtgttccttgcctcgctgggcccatggggaacagtgagcaggccgctctctgtgggtagtaggatggggttatcagctggggctggtccaggggaggggctgctgctacattccgggccagactggcccacgcggaaagagaacttgggctggtccgagccacagccgtcttcaatgccatctactaccctggggctcagatctgggggcacattccatggcatggggggcagccgtagcccctctagggcccgtgggggagcagaggggccagcctcagccttcaaagcccctgccctgcctggcctccctctgccacctagacgaggccggggtgctgttcgacgtggggatagcagcttggcagctgaggatgaggaggtgcagccaggggacagcagggggctggagggctcatcagctggggctggggagaccgtggggccctgctccccatctgtctccttctcctccagcgtggacataagggtattgtcgccgctcagggagctggtgtccacctctgcagagcctcccccagcacccaggttgtagctgagctcccctcggaggccacgactgaagcgcggggcaaactcggggtacagcgcaaggctgtcgtgcaggccagccagctgcagacactgcaggacgcagtacgtcagccccttcacgtcggcattggcctttaccacctgctcccgccggggcagctcacagccgatcaggtcgcccttccctaggatggcgagcacggtgccacccttgagcacctccatggagccagagcagacaaagtagagggcctgcagggcatcgccttggtggatgaggtactcgcccggcgtgcagaaggcgggccgcagggccagagacagtgcccgcaggcagccgcggctggccgcctcaaacagtggcagctgcaggacctccttgtgcaggtgcatggcgatgtctgcgcgcagctcgtcagggaggctctgcagcagctcggtggtgtcgatgccattgttcaccgcccaggtggcctggaagtactccagcatgcgctgcttgaggggcttggggatacggtggatgcggatgtagtcgcgcaggtcgcgcgtgcggctgtggtacagaaagcggcgggcgtacatgcgctggatgatggccgtcacgttcccaaacaccaccgcgtgcatcagggcgccgatgagcatggtgcagatggagaagatcttctcggtgtccgtgttggcggacacgttgccgaagcccacgctggtgaggctgctgagtgcgaagtagagggaggtgatgtaggcgctgcgcagcgacgggccgcccagcagctccagccccgtcccgttggcctcgctgctgctgctgcagttgtcactctggccggagctgttccctccagctggcctccggcccaccaggtagtagggagtctccagtcggcgggccagctcctgcagccagccaatctcaggcagctcggattcgctgctctcgatctcccgctggccaatgtaaaaccagacgcaggcgacccagtgcgcgagcagggcgaacacggccatgagcagtgtcagcaccacggcgctgtactgcgagtaccggtccagccgcggaagcaggcgcagcaggcgcagcaggcgcaccgtcttcagcagatgggccccgaagtacacgttgaccttgaaggcatgtagcaggtcaaagggcagcgctgcgatgacatccagcaggaaccaggtggtgacgtagtggaggcaaatggactttggggcaaacaccacctggcccgacttggacacgaatgtggtacggaaattcagcacaatgtcaaggatgaagaggacctccacggccaggtcacagacgctgggcgggccgcgggcggcactgggctcccgtgctgtgctcacacacacgctgtagggcacagtgacagccacatagagtgtggcgagcaggatgaagccatcccaggtggctctcagtgccccacagtgcaacaggatgaagggcgacttccggatggcggctactttgtactcaggcaagtttggtttctccccaaacacccccttattgagcttgtgcttgcccttgggctgcttctgcaggtgcccggacaggtggtagagcacggcccggctccgccgccggttggcattgaagcctttggatcgtgcccggccatatcggcgccggccaccacctgtctccttccatctgtcggggccccctcggttcttggtttcgctgatgtccttgtgagagactaggaagagagccacctcccctttctcattctttatgggtatcacatccaggagacaccagaacgggagccgcgtgccgtcgaagcgcgtagcgatggtgtccaggaaggtgttctgcggcgccaggaggccccgcatggccggcatcttaggcgcccgcggctgcccgccccatccctccggggtgcggggactccgcgccgggggagggcgcccagctcggccgccccccgccgggccccgcgctccctagcgcagccgtcggggggcaatgcgcagaccgggatccggggtcgcgccggacgctggcgcgcgagggggcgtccgcgccgtcggggcccggagcatggcgcgcggcccctcgcgccctcgccgcccacaaatcccgggctccaggccccgcggccgccgcgctctcagcacctcccgccgcggcagcggctcgcgtgtcggctgcgggtgggcttccgctcggcttcgctcggcgccggctctcggcagctccctccgtctgtcggggagaagctgcagcctccctccctccctcccgcgcccgccgcctgcaccggggtaaccatggagacggggcacacccagccagggccgcctccttaaagggacaggcctcccgcggagggctcccctcccttcgggacctcggcgggggcggggaggtggcggccgccctgatcccaccccgcgggcctccccgcccgtacctcggagaaccactggcgagcggccggccccctttggctcactcggcctcagccgcagaggggaggcgtctttctctgcagcccgggggctctccgagagcctcctagcagcctctcctcccccggcggaatgggaggggggctcggggcgtggggggcaggggacgcatgctgtggaagatgctctccccgaggaaaatgcagtgggcaaggggacagggcgacaggcgcaggtgaaggccctgcggccagcggaggccggcgctctagaggggctccagccgcacccgggaaatctaaaagc

SEQ ID NO: 10767 - RNA, 4436 nt, Homo sapiens
  source 1..4436: mol_type = other RNA
ctcccctctctttcctgttcagcaaaagaaatttggctcaggatggatgaagggggaaataggcaaatactacttctccaggtaaccagtagccgagcagcctccgccagctgtcttttgtgccagcttggctgttgaagcccaagtaactggcagagactcctgccatgccattctccttcaaacctctgtcatctgcttgcccacaaatgtcctcgtcccattctccatgcaagcattggtcctctggcaaattcacaccaacataattccaaactgcacatctatttccacattctctcatcagtaaattgctttgtcactttgccaatgacttagcagcaatagggctccccagctacctattgcttccctcatcatccctcgccctctagagttcctttggagggttcagaatgaatcaagggtccagtggagatcctatttcctttatcatcccctccatgtctggagaatagaatggtatcaggatgctctttaggggcacaattaggaagacttttcctcctctctcctcacacctttctggcctcagaaccagtcctctctttcaggtcttccctccatccctgagagaccctggtagtatcaaagtctctaaggtatggtggaaagagataaggagtcacactagtagttgtgggaagcaggctggctcctgtaagctgtctgtagggtaatgaaaggaggactttgcccacagtaggggctctacacatgatggttggctggttcctaggatgggtgaaagaacataaaggccacaagttctgtgggtcccagaggcctgctgctccaacattgtgccaggaagattcttctgaacacaagagctctaaggctgttcgctgttttccaaagaaatgtctgactctttttgccacagagcccctggcagccgagaggacgggtattaccatcgaggaatgaaatcaggcatctctgggtttctccccggaactctcaaggatttcagttcccaattaccacttttattggttctctctagacctcaaattccacacaatgctgtggtgtaatggaacagctttggagtcagacctggctgaagctccaggtctgcggcttaaactggtcaaaacactctgagagtgctacctctctgagcctcatctaaacaatgatgtttgtcatattatcagccttgccttcttcaaaggagataatacaagagaaattattttccaaacatgaaggagtggttcttgttggtttctgctacaactgcggactgtccgaggcactttataggagttagggccagacacatgcctggagttcacctcaccttgggttgcaaggctgtcattagcaaccagacaacggaggcctagcccatcacgtctcaccctgacccttgaagggccaagcagtgtggttgcttagaaagggaaggcacagctgagaaataagtacccgctgttcttggtgaatttcagctgcctgaaggaaattattccccatctcctgaaaaggaaacacatttcaggaacaagaggagcagactgtacaaggctggccttcccaggtttgggctggatctagcacccagaaaccaggctgagcccaggcactttgaagtaaggctctcgagggtcctaccatatgatctgttgggaagcttggggtttaggggaaggtgaatttggacctgaactagggggcagatccctgctcagtgcctagacactggcttctcctgagcctggctttaggggagcagcatgagcacctgcggtgacaatgctctgctgtggctttttgaagccagagtgaagaaagactgggttagtacagcatcagctgctggcctttcagataaggcctggcctaacgtccacttgggttgcagcaaacttgaacaaaatccctctgtcctatcctcaccccttgccctttctaggccaggtaaaaaggctctgccttgctaatgcccaggagcagtctaggatttgggaatttagaaggctgtggtgagggctaagagtcacaggtactagaaattgaagggacttctggaggtcatcccgtccaacccttcgtccccagacagaatttgattaggaatggatgaaaaacatttgtactgcttaataaatggaaaattctgtttgtgcccaggtaagctaaagaatatcccagactcacatgaccacaggtcccaggttaggcacctgtctcagacagaggtaggctccatggagaaagaagacaggagttctagtcaggctgggaatgggggcaactagaaggtgaccccagggaattttctgagtgtggagcacagctgtaaataaaatgagagtcatgtgacccaagtacggattcagggtcttaggcgggcaggtttgtggccattccctgtgattgttccaaagcacagcaaacttcccaaagcccagcaagctgccacggtgtggctgtcagctggagtgggaagagcactccaaccctcctgcaggccacagtatagagcagaaagaacattcccactgccaaggatgctccttggcaggtttctcttatggtctctgccaaaagcacctgccttttccctctctggccttcttcttaggctgcaatgctcccttcccactccaccccagccactaccctacccaagagaggagcagcagcccccttggggtcagatgtccacccccagagtctggagtgcacctttgctttctctggcctgctgccctggatcctcattttagtgcaacaaacaatagatctgacaacagggacctcggggttgaagagtcatgccataagtcagtcaacatggaaccaaagaaggttctgcttcatgtaaaccctggggctccatcaactgtcctgttaactcaaggtcattctggaaagtcaagcaggccttgtcaccctggagtcactggggaataaataacactggggcatttctctgcggctgcaacaccaatacacctcactccacagcagcacttagaggttctgggagtcctggctcccaaacccagggaaggggcacggacagaggcaaaatggggggaatctaggatgcaggggcttcacccagcctgatggccccaaagaacgtggtgtgcttgctcatgttgatggagatgtcagcgtgcaccatcttgacggcgatcttctgccgggccttgaggaggcagacgcctgcggtatagcaagtgttgtagttggtcttgcccgtctcgatgctgcgtgtgcactgcaggaagggcttctcatccaccaccacctcatagctggcaaagtcagtgaagttgatgtagtatacctccagctccccgctgcggggatgtagcttaaacaccttggggttcatagtgatgcgagaccagtcattgagcactccacctgaaagatcattcttgacttgaattgctgacccttggccctgtagatgcaccacagctggctggttttctcgagttccagctttatcagcagcaccagaaggtccctggaggccagggggtccttgaggaccaggaggacctggaggaccaggtggtcccataacagttgttcctggaattccaggaatccctggaattcctgggggtccctggggtcctggaggtcctgggggtcctggagggccattgggtccaggaggtcctgctttctttccctttttcttgtttttaactgggccatctgctccttcattgcttttgcttcttttattgcggcgaacacgcctactttcttcttcagagtatggcttttcatcagggaagaagaaattcaatagggccatctggtgcccgtcctgggagtcagagtggagtgcggcttctcccggttccaatggctgctgcttaggtgacggctgcccaaggtgactggtgatggggctgtcagggtcgaggccaccgaggctgcttagggtgccagaggtgccaggggtgcccgagccgccaaggcgggactcggctccacgttcccgccgcaactccgagcgcaactctaggtagcagcacaacgtcagcaggtggagggccagcgagaggccaaagaaacccaggaagagcaggcagctgttcccttcgcccgcccgggcaggggccccgccacacccgcagccctggctccctcgctcccgcggcgctgctgcaggcaggagttccctgcgctccacctccgggtagcccatggcctccggagacacccactctcttgaggcccgggagccgctgcgtctgcctcagccgttcacgacctctgacaggcggctactgtcctgccatcggctgggggctgcagggacccgttcctgcgcgacagtggctgggcgggacggagcagggagcagccgcatgtgcagctctactccgaggggtgggaaagggaggaggaggggcgggagagaggggagg

SEQ ID NO: 10768 - RNA, 4436 nt, Homo sapiens
  source 1..4436: mol_type = other RNA
ctcccctctctttcctgttcagcaaaagaaatttggctcaggatggatgaagggggaaataggcaaatactacttctccaggtaaccagtagccgagcagcctccgccagctgtcttttgtgccagcttggctgttgaagcccaagtaactggcagagactcctgccatgccattctccttcaaacctctgtcatctgcttgcccacaaatgtcctcgtcccattctccatgcaagcattggtcctctggcaaattcacaccaacataattccaaactgcacatctatttccacattctctcatcagtaaattgctttgtcactttgccaatgacttagcagcaatagggctccccagctacctattgcttccctcatcatccctcgccctctagagttcctttggagggttcagaatgaatcaagggtccagtggagatcctatttcctttatcatcccctccatgtctggagaatagaatggtatcaggatgctctttaggggcacaattaggaagacttttcctcctctctcctcacacctttctggcctcagaaccagtcctctctttcaggtcttccctccatccctgagagaccctggtagtatcaaagtctctaaggtatggtggaaagagataaggagtcacactagtagttgtgggaagcaggctggctcctgtaagctgtctgtagggtaatgaaaggaggactttgcccacagtaggggctctacacatgatggttggctggttcctaggatgggtgaaagaacataaaggccacaagttctgtgggtcccagaggcctgctgctccaacattgtgccaggaagattcttctgaacacaagagctctaaggctgttcgctgttttccaaagaaatgtctgactctttttgccacagagcccctggcagccgagaggacgggtattaccatcgaggaatgaaatcaggcatctctgggtttctccccggaactctcaaggatttcagttcccaattaccacttttattggttctctctagacctcaaattccacacaatgctgtggtgtaatggaacagctttggagtcagacctggctgaagctccaggtctgcggcttaaactggtcaaaacactctgagagtgctacctctctgagcctcatctaaacaatgatgtttgtcatattatcagccttgccttcttcaaaggagataatacaagagaaattattttccaaacatgaaggagtggttcttgttggtttctgctacaactgcggactgtccgaggcactttataggagttagggccagacacatgcctggagttcacctcaccttgggttgcaaggctgtcattagcaaccagacaacggaggcctagcccatcacgtctcaccctgacccttgaagggccaagcagtgtggttgcttagaaagggaaggcacagctgagaaataagtacccgctgttcttggtgaatttcagctgcctgaaggaaattattccccatctcctgaaaaggaaacacatttcaggaacaagaggagcagactgtacaaggctggccttcccaggtttgggctggatctagcacccagaaaccaggctgagcccaggcactttgaagtaaggctctcgagggtcctaccatatgatctgttgggaagcttggggtttaggggaaggtgaatttggacctgaactagggggcagatccctgctcagtgcctagacactggcttctcctgagcctggctttaggggagcagcatgagcacctgcggtgacaatgctctgctgtggctttttgaagccagagtgaagaaagactgggttagtacagcatcagctgctggcctttcagataaggcctggcctaacgtccacttgggttgcagcaaacttgaacaaaatccctctgtcctatcctcaccccttgccctttctaggccaggtaaaaaggctctgccttgctaatgcccaggagcagtctaggatttgggaatttagaaggctgtggtgagggctaagagtcacaggtactagaaattgaagggacttctggaggtcatcccgtccaacccttcgtccccagacagaatttgattaggaatggatgaaaaacatttgtactgcttaataaatggaaaattctgtttgtgcccaggtaagctaaagaatatcccagactcacatgaccacaggtcccaggttaggcacctgtctcagacagaggtaggctccatggagaaagaagacaggagttctagtcaggctgggaatgggggcaactagaaggtgaccccagggaattttctgagtgtggagcacagctgtaaataaaatgagagtcatgtgacccaagtacggattcagggtcttaggcgggcaggtttgtggccattccctgtgattgttccaaagcacagcaaacttcccaaagcccagcaagctgccacggtgtggctgtcagctggagtgggaagagcactccaaccctcctgcaggccacagtatagagcagaaagaacattcccactgccaaggatgctccttggcaggtttctcttatggtctctgccaaaagcacctgccttttccctctctggccttcttcttaggctgcaatgctcccttcccactccaccccagccactaccctacccaagagaggagcagcagcccccttggggtcagatgtccacccccagagtctggagtgcacctttgctttctctggcctgctgccctggatcctcattttagtgcaacaaacaatagatctgacaacagggacctcggggttgaagagtcatgccataagtcagtcaacatggaaccaaagaaggttctgcttcatgtaaaccctggggctccatcaactgtcctgttaactcaaggtcattctggaaagtcaagcaggccttgtcaccctggagtcactggggaataaataacactggggcatttctctgcggctgcaacaccaatacacctcactccacagcagcacttagaggttctgggagtcctggctcccaaacccagggaaggggcacggacagaggcaaaatggggggaatctaggatgcaggggcttcacccagcctgatggccccaaagaacgtggtgtgcttgctcatgttgatggagatgtcagcgtgcaccatcttgacggcgatcttctgccgggccttgaggaggcagacgcctgcggtatagcaagtgttgtagttggtcttgcccgtctcgatgctgcgtgtgcactgcaggaagggcttctcatccaccaccacctcatagctggcaaagtcagtgaagttgatgtagtatacctgactatagatgaagtaggtgccgtccaccagtacctccagctccccgctgcggggatgtagcttaaacaccttggggttcatagtgatgcgagaccagtcattgagcactccaccattcttgacttgaattgctgacccttggccctgtagatgcaccacagctggctggttttctcgagttccagctttatcagcagcaccagaaggtccctggaggccagggggtccttgaggaccaggaggacctggaggaccaggtggtcccataacagttgttcctggaattccaggaatccctggaattcctgggggtccctggggtcctggaggtcctgggggtcctggagggccattgggtccaggaggtcctgctttctttccctttttcttgtttttaactgggccatctgctccttcattgcttttgcttcttttattgcggcgaacacgcctactttcttcttcagagtatggcttttcatcagggaagaagaaattcaatagggccatctggtgcccgtcctgggagtcagagtggagtgcggcttctcccggttccaatggctgctgcttaggtgacggctgcccaaggtgactggtgatggggctgtcagggtcgaggccaccgaggctgcttagggtgccagaggtgccaggggtgcccgagccgccaaggcgggactcggctccacgttcccgccgcaactccgagcgcaactctaggtagcagcacaacgtcagcaggtggagggccagcgagaggccaaagaaacccaggaagagcaggcagctgttcccttcgcccgcccgggcaggggccccgccacacccgcagccctggctccctcgctcccgcggcgctgctgcaggcaggagttccctgcgctccacctccgggtagcccatggcctccggagacacccactctcttgaggcccgggagccgctgcgtctgcctcagccgttcacgacctctgacaggcggctactgtcctgccatcggctgggggctgcagggacccgttcctgcgcgacagtggctgggcgggacggagcagggagcagccgcatgtgcagctctactccgaggggtgggaaaggg

SEQ ID NO: 10769 - RNA, 4445 nt, Homo sapiens
  source 1..4445: mol_type = other RNA
ctcccctctctttcctgttcagcaaaagaaatttggctcaggatggatgaagggggaaataggcaaatactacttctccaggtaaccagtagccgagcagcctccgccagctgtcttttgtgccagcttggctgttgaagcccaagtaactggcagagactcctgccatgccattctccttcaaacctctgtcatctgcttgcccacaaatgtcctcgtcccattctccatgcaagcattggtcctctggcaaattcacaccaacataattccaaactgcacatctatttccacattctctcatcagtaaattgctttgtcactttgccaatgacttagcagcaatagggctccccagctacctattgcttccctcatcatccctcgccctctagagttcctttggagggttcagaatgaatcaagggtccagtggagatcctatttcctttatcatcccctccatgtctggagaatagaatggtatcaggatgctctttaggggcacaattaggaagacttttcctcctctctcctcacacctttctggcctcagaaccagtcctctctttcaggtcttccctccatccctgagagaccctggtagtatcaaagtctctaaggtatggtggaaagagataaggagtcacactagtagttgtgggaagcaggctggctcctgtaagctgtctgtagggtaatgaaaggaggactttgcccacagtaggggctctacacatgatggttggctggttcctaggatgggtgaaagaacataaaggccacaagttctgtgggtcccagaggcctgctgctccaacattgtgccaggaagattcttctgaacacaagagctctaaggctgttcgctgttttccaaagaaatgtctgactctttttgccacagagcccctggcagccgagaggacgggtattaccatcgaggaatgaaatcaggcatctctgggtttctccccggaactctcaaggatttcagttcccaattaccacttttattggttctctctagacctcaaattccacacaatgctgtggtgtaatggaacagctttggagtcagacctggctgaagctccaggtctgcggcttaaactggtcaaaacactctgagagtgctacctctctgagcctcatctaaacaatgatgtttgtcatattatcagccttgccttcttcaaaggagataatacaagagaaattattttccaaacatgaaggagtggttcttgttggtttctgctacaactgcggactgtccgaggcactttataggagttagggccagacacatgcctggagttcacctcaccttgggttgcaaggctgtcattagcaaccagacaacggaggcctagcccatcacgtctcaccctgacccttgaagggccaagcagtgtggttgcttagaaagggaaggcacagctgagaaataagtacccgctgttcttggtgaatttcagctgcctgaaggaaattattccccatctcctgaaaaggaaacacatttcaggaacaagaggagcagactgtacaaggctggccttcccaggtttgggctggatctagcacccagaaaccaggctgagcccaggcactttgaagtaaggctctcgagggtcctaccatatgatctgttgggaagcttggggtttaggggaaggtgaatttggacctgaactagggggcagatccctgctcagtgcctagacactggcttctcctgagcctggctttaggggagcagcatgagcacctgcggtgacaatgctctgctgtggctttttgaagccagagtgaagaaagactgggttagtacagcatcagctgctggcctttcagataaggcctggcctaacgtccacttgggttgcagcaaacttgaacaaaatccctctgtcctatcctcaccccttgccctttctaggccaggtaaaaaggctctgccttgctaatgcccaggagcagtctaggatttgggaatttagaaggctgtggtgagggctaagagtcacaggtactagaaattgaagggacttctggaggtcatcccgtccaacccttcgtccccagacagaatttgattaggaatggatgaaaaacatttgtactgcttaataaatggaaaattctgtttgtgcccaggtaagctaaagaatatcccagactcacatgaccacaggtcccaggttaggcacctgtctcagacagaggtaggctccatggagaaagaagacaggagttctagtcaggctgggaatgggggcaactagaaggtgaccccagggaattttctgagtgtggagcacagctgtaaataaaatgagagtcatgtgacccaagtacggattcagggtcttaggcgggcaggtttgtggccattccctgtgattgttccaaagcacagcaaacttcccaaagcccagcaagctgccacggtgtggctgtcagctggagtgggaagagcactccaaccctcctgcaggccacagtatagagcagaaagaacattcccactgccaaggatgctccttggcaggtttctcttatggtctctgccaaaagcacctgccttttccctctctggccttcttcttaggctgcaatgctcccttcccactccaccccagccactaccctacccaagagaggagcagcagcccccttggggtcagatgtccacccccagagtctggagtgcacctttgctttctctggcctgctgccctggatcctcattttagtgcaacaaacaatagatctgacaacagggacctcggggttgaagagtcatgccataagtcagtcaacatggaaccaaagaaggttctgcttcatgtaaaccctggggctccatcaactgtcctgttaactcaaggtcattctggaaagtcaagcaggccttgtcaccctggagtcactggggaataaataacactggggcatttctctgcggctgcaacaccaatacacctcactccacagcagcacttagaggttctgggagtcctggctcccaaacccagggaaggggcacggacagaggcaaaatggggggaatctaggatgcaggggcttcacccagcctgatggccccaaagaacgtggtgtgcttgctcatgttgatggagatgtcagcgtgcaccatcttgacggcgatcttctgccgggccttgaggaggcagacgcctgcggtatagcaagtgttgtagttggtcttgcccgtctcgatgctgcgtgtgcactgcaggaagggcttctcatccaccaccacctcatagctggcaaagtcagtgaagttgatgtagtatacctgactatagatgaagtaggtgccgtccaccagtacctccagctccccgctgcggggatgtagcttaaacaccttggggttcatagtgatgcgagaccagtcattgagcactccacctgaaagatcattcttgacttgaattgctgacccttggccctgtagatgcaccacagctggctggttttctcgagttccagctttatcagcagcaccagaaggtccctggaggccagggggtccttgaggaccaggaggacctggaggaccaggtggtcccataacagttgttcctggaattccaggaatccctggaattcctgggggtccctggggtcctggaggtcctgggggtcctggagggccattgggtccaggaggtcctgctttctttccctttttcttgtttttaactgggccatctgctccttcattgcttttgcttcttttattgcggcgaacacgcctactttcttcttcagagtatggcttttcatcagggaagaagaaattcaatagggccatctggtgcccgtcctgggagtcagagtggagtgcggcttctcccggttccaatggctgctgcttaggtgacggctgcccaaggtgactggtgatggggctgtcagggtcgaggccaccgaggctgcttagggtgccagaggtgccaggggtgcccgagccgccaaggcgggactcggctccacgttcccgccgcaactccgagcgcaactctaggtagcagcacaacgtcagcaggtggagggccagcgagaggccaaagaaacccaggaagagcaggcagctgttcccttcgcccgcccgggcaggggccccgccacacccgcagccctggctccctcgctcccgcggcgctgctgcaggcaggagttccctgcgctccacctccgggtagcccatggcctccggagacacccactctcttgaggcccgggagccgctgcgtctgcctcagccgttcacgacctctgacaggcggctactgtcctgccatcggctgggggctgcagggacccgttcctgcgcgacagtggctgggcgggacggagcagggagcagccgcatgtgcagctctactccgaggggtgggaaaggg

SEQ ID NO: 10770 - RNA, 4469 nt, Homo sapiens
  source 1..4469: mol_type = other RNA
ctcccctctctttcctgttcagcaaaagaaatttggctcaggatggatgaagggggaaataggcaaatactacttctccaggtaaccagtagccgagcagcctccgccagctgtcttttgtgccagcttggctgttgaagcccaagtaactggcagagactcctgccatgccattctccttcaaacctctgtcatctgcttgcccacaaatgtcctcgtcccattctccatgcaagcattggtcctctggcaaattcacaccaacataattccaaactgcacatctatttccacattctctcatcagtaaattgctttgtcactttgccaatgacttagcagcaatagggctccccagctacctattgcttccctcatcatccctcgccctctagagttcctttggagggttcagaatgaatcaagggtccagtggagatcctatttcctttatcatcccctccatgtctggagaatagaatggtatcaggatgctctttaggggcacaattaggaagacttttcctcctctctcctcacacctttctggcctcagaaccagtcctctctttcaggtcttccctccatccctgagagaccctggtagtatcaaagtctctaaggtatggtggaaagagataaggagtcacactagtagttgtgggaagcaggctggctcctgtaagctgtctgtagggtaatgaaaggaggactttgcccacagtaggggctctacacatgatggttggctggttcctaggatgggtgaaagaacataaaggccacaagttctgtgggtcccagaggcctgctgctccaacattgtgccaggaagattcttctgaacacaagagctctaaggctgttcgctgttttccaaagaaatgtctgactctttttgccacagagcccctggcagccgagaggacgggtattaccatcgaggaatgaaatcaggcatctctgggtttctccccggaactctcaaggatttcagttcccaattaccacttttattggttctctctagacctcaaattccacacaatgctgtggtgtaatggaacagctttggagtcagacctggctgaagctccaggtctgcggcttaaactggtcaaaacactctgagagtgctacctctctgagcctcatctaaacaatgatgtttgtcatattatcagccttgccttcttcaaaggagataatacaagagaaattattttccaaacatgaaggagtggttcttgttggtttctgctacaactgcggactgtccgaggcactttataggagttagggccagacacatgcctggagttcacctcaccttgggttgcaaggctgtcattagcaaccagacaacggaggcctagcccatcacgtctcaccctgacccttgaagggccaagcagtgtggttgcttagaaagggaaggcacagctgagaaataagtacccgctgttcttggtgaatttcagctgcctgaaggaaattattccccatctcctgaaaaggaaacacatttcaggaacaagaggagcagactgtacaaggctggccttcccaggtttgggctggatctagcacccagaaaccaggctgagcccaggcactttgaagtaaggctctcgagggtcctaccatatgatctgttgggaagcttggggtttaggggaaggtgaatttggacctgaactagggggcagatccctgctcagtgcctagacactggcttctcctgagcctggctttaggggagcagcatgagcacctgcggtgacaatgctctgctgtggctttttgaagccagagtgaagaaagactgggttagtacagcatcagctgctggcctttcagataaggcctggcctaacgtccacttgggttgcagcaaacttgaacaaaatccctctgtcctatcctcaccccttgccctttctaggccaggtaaaaaggctctgccttgctaatgcccaggagcagtctaggatttgggaatttagaaggctgtggtgagggctaagagtcacaggtactagaaattgaagggacttctggaggtcatcccgtccaacccttcgtccccagacagaatttgattaggaatggatgaaaaacatttgtactgcttaataaatggaaaattctgtttgtgcccaggtaagctaaagaatatcccagactcacatgaccacaggtcccaggttaggcacctgtctcagacagaggtaggctccatggagaaagaagacaggagttctagtcaggctgggaatgggggcaactagaaggtgaccccagggaattttctgagtgtggagcacagctgtaaataaaatgagagtcatgtgacccaagtacggattcagggtcttaggcgggcaggtttgtggccattccctgtgattgttccaaagcacagcaaacttcccaaagcccagcaagctgccacggtgtggctgtcagctggagtgggaagagcactccaaccctcctgcaggccacagtatagagcagaaagaacattcccactgccaaggatgctccttggcaggtttctcttatggtctctgccaaaagcacctgccttttccctctctggccttcttcttaggctgcaatgctcccttcccactccaccccagccactaccctacccaagagaggagcagcagcccccttggggtcagatgtccacccccagagtctggagtgcacctttgctttctctggcctgctgccctggatcctcattttagtgcaacaaacaatagatctgacaacagggacctcggggttgaagagtcatgccataagtcagtcaacatggaaccaaagaaggttctgcttcatgtaaaccctggggctccatcaactgtcctgttaactcaaggtcattctggaaagtcaagcaggccttgtcaccctggagtcactggggaataaataacactggggcatttctctgcggctgcaacaccaatacacctcactccacagcagcacttagaggttctgggagtcctggctcccaaacccagggaaggggcacggacagaggcaaaatggggggaatctaggatgcaggggcttcacccagcctgatggccccaaagaacgtggtgtgcttgctcatgttgatggagatgtcagcgtgcaccatcttgacggcgatcttctgccgggccttgaggaggcagacgcctgcggtatagcaagtgttgtagttggtcttgcccgtctcgatgctgcgtgtgcactgcaggaagggcttctcatccaccaccacctcatagctggcaaagtcagtgaagttgatgtagtatacttctacctgactatagatgaagtaggtgccgtccaccagtacctccagctccccgctgcggggatgtagcttaaacaccttggggttcatagtgatgcgagaccagtcattgagcactccaccattcttgacttgaattgctgacccttggccctgtagatgcaccacagctggctggttttctcgagttccagctttatcagcagcaccagaaggtccctggaggccagggggtccttgaggaccaggaggacctggaggaccaggtggtcccataacagttgttcctggaattccaggaatccctggaattcctgggggtccctggggtcctggaggtcctgggggtcctggagggccattgggtccaggaggtcctgctttctttccctttttcttgtttttaactgggccatctgctccttcattgcttttgcttcttttattgcggcgaacacgcctactttcttcttcagagtatggcttttcatcagggaagaagaaattcaatagggccatctggtgcccgtcctgggagtcagagtggagtgcggcttctcccggttccaatggctgctgcttaggtgacggctgcccaaggtgactggtgatggggctgtcagggtcgaggccaccgaggctgcttagggtgccagaggtgccaggggtgcccgagccgccaaggcgggactcggctccacgttcccgccgcaactccgagcgcaactctaggtagcagcacaacgtcagcaggtggagggccagcgagaggccaaagaaacccaggaagagcaggcagctgttcccttcgcccgcccgggcaggggccccgccacacccgcagccctggctccctcgctcccgcggcgctgctgcaggcaggagttccctgcgctccacctccgggtagcccatggcctccggagacacccactctcttgaggcccgggagccgctgcgtctgcctcagccgttcacgacctctgacaggcggctactgtcctgccatcggctgggggctgcagggacccgttcctgcgcgacagtggctgggcgggacggagcagggagcagccgcatgtgcagctctactccgaggggtgggaaagggaggaggaggggcgggagagaggggagg

SEQ ID NO: 10771 - RNA, 4451 nt, Homo sapiens
  source 1..4451: mol_type = other RNA
ctcccctctctttcctgttcagcaaaagaaatttggctcaggatggatgaagggggaaataggcaaatactacttctccaggtaaccagtagccgagcagcctccgccagctgtcttttgtgccagcttggctgttgaagcccaagtaactggcagagactcctgccatgccattctccttcaaacctctgtcatctgcttgcccacaaatgtcctcgtcccattctccatgcaagcattggtcctctggcaaattcacaccaacataattccaaactgcacatctatttccacattctctcatcagtaaattgctttgtcactttgccaatgacttagcagcaatagggctccccagctacctattgcttccctcatcatccctcgccctctagagttcctttggagggttcagaatgaatcaagggtccagtggagatcctatttcctttatcatcccctccatgtctggagaatagaatggtatcaggatgctctttaggggcacaattaggaagacttttcctcctctctcctcacacctttctggcctcagaaccagtcctctctttcaggtcttccctccatccctgagagaccctggtagtatcaaagtctctaaggtatggtggaaagagataaggagtcacactagtagttgtgggaagcaggctggctcctgtaagctgtctgtagggtaatgaaaggaggactttgcccacagtaggggctctacacatgatggttggctggttcctaggatgggtgaaagaacataaaggccacaagttctgtgggtcccagaggcctgctgctccaacattgtgccaggaagattcttctgaacacaagagctctaaggctgttcgctgttttccaaagaaatgtctgactctttttgccacagagcccctggcagccgagaggacgggtattaccatcgaggaatgaaatcaggcatctctgggtttctccccggaactctcaaggatttcagttcccaattaccacttttattggttctctctagacctcaaattccacacaatgctgtggtgtaatggaacagctttggagtcagacctggctgaagctccaggtctgcggcttaaactggtcaaaacactctgagagtgctacctctctgagcctcatctaaacaatgatgtttgtcatattatcagccttgccttcttcaaaggagataatacaagagaaattattttccaaacatgaaggagtggttcttgttggtttctgctacaactgcggactgtccgaggcactttataggagttagggccagacacatgcctggagttcacctcaccttgggttgcaaggctgtcattagcaaccagacaacggaggcctagcccatcacgtctcaccctgacccttgaagggccaagcagtgtggttgcttagaaagggaaggcacagctgagaaataagtacccgctgttcttggtgaatttcagctgcctgaaggaaattattccccatctcctgaaaaggaaacacatttcaggaacaagaggagcagactgtacaaggctggccttcccaggtttgggctggatctagcacccagaaaccaggctgagcccaggcactttgaagtaaggctctcgagggtcctaccatatgatctgttgggaagcttggggtttaggggaaggtgaatttggacctgaactagggggcagatccctgctcagtgcctagacactggcttctcctgagcctggctttaggggagcagcatgagcacctgcggtgacaatgctctgctgtggctttttgaagccagagtgaagaaagactgggttagtacagcatcagctgctggcctttcagataaggcctggcctaacgtccacttgggttgcagcaaacttgaacaaaatccctctgtcctatcctcaccccttgccctttctaggccaggtaaaaaggctctgccttgctaatgcccaggagcagtctaggatttgggaatttagaaggctgtggtgagggctaagagtcacaggtactagaaattgaagggacttctggaggtcatcccgtccaacccttcgtccccagacagaatttgattaggaatggatgaaaaacatttgtactgcttaataaatggaaaattctgtttgtgcccaggtaagctaaagaatatcccagactcacatgaccacaggtcccaggttaggcacctgtctcagacagaggtaggctccatggagaaagaagacaggagttctagtcaggctgggaatgggggcaactagaaggtgaccccagggaattttctgagtgtggagcacagctgtaaataaaatgagagtcatgtgacccaagtacggattcagggtcttaggcgggcaggtttgtggccattccctgtgattgttccaaagcacagcaaacttcccaaagcccagcaagctgccacggtgtggctgtcagctggagtgggaagagcactccaaccctcctgcaggccacagtatagagcagaaagaacattcccactgccaaggatgctccttggcaggtttctcttatggtctctgccaaaagcacctgccttttccctctctggccttcttcttaggctgcaatgctcccttcccactccaccccagccactaccctacccaagagaggagcagcagcccccttggggtcagatgtccacccccagagtctggagtgcacctttgctttctctggcctgctgccctggatcctcattttagtgcaacaaacaatagatctgacaacagggacctcggggttgaagagtcatgccataagtcagtcaacatggaaccaaagaaggttctgcttcatgtaaaccctggggctccatcaactgtcctgttaactcaaggtcattctggaaagtcaagcaggccttgtcaccctggagtcactggggaataaataacactggggcatttctctgcggctgcaacaccaatacacctcactccacagcagcacttagaggttctgggagtcctggctcccaaacccagggaaggggcacggacagaggcaaaatggggggaatctaggatgcaggggcttcacccagcctgatggccccaaagaacgtggtgtgcttgctcatgttgatggagatgtcagcgtgcaccatcttgacggcgatcttctgccgggccttgaggaggcagacgcctgcggtatagcaagtgttgtagttggtcttgcccgtctcgatgctgcgtgtgcactgcaggaagggcttctcatccaccaccacctcatagctggcaaagtcagtgaagttgatgtagtatacttctacctgactatagatgaagtaggtgccgtccaccagtacctccagctccccgctgcggggatgtagcttaaacaccttggggttcatagtgatgcgagaccagtcattgagcactccacctgaaagatcattcttgacttgaattgctgacccttggccctgtagatgcaccacagctggctggttttctcgagttccagctttatcagcagcaccagaaggtccctggaggccagggggtccttgaggaccaggaggacctggaggaccaggtggtcccataacagttgttcctggaattccaggaatccctggaattcctgggggtccctggggtcctggaggtcctgggggtcctggagggccattgggtccaggaggtcctgctttctttccctttttcttgtttttaactgggccatctgctccttcattgcttttgcttcttttattgcggcgaacacgcctactttcttcttcagagtatggcttttcatcagggaagaagaaattcaatagggccatctggtgcccgtcctgggagtcagagtggagtgcggcttctcccggttccaatggctgctgcttaggtgacggctgcccaaggtgactggtgatggggctgtcagggtcgaggccaccgaggctgcttagggtgccagaggtgccaggggtgcccgagccgccaaggcgggactcggctccacgttcccgccgcaactccgagcgcaactctaggtagcagcacaacgtcagcaggtggagggccagcgagaggccaaagaaacccaggaagagcaggcagctgttcccttcgcccgcccgggcaggggccccgccacacccgcagccctggctccctcgctcccgcggcgctgctgcaggcaggagttccctgcgctccacctccgggtagcccatggcctccggagacacccactctcttgaggcccgggagccgctgcgtctgcctcagccgttcacgacctctgacaggcggctactgtcctgccatcggctgggggctgcagggacccgttcctgcgcgacagtggctgggcgggacggagcagggagcagccgcatgtgcagctctactccgaggggtgggaaaggg

SEQ ID NO: 10772 - RNA, 49 nt, Homo sapiens
  source 1..49: mol_type = other RNA
ctccgggacggctgggcgccggcggccgggagatccgcgcttcctgaat

SEQ ID NO: 10773 - RNA, 117 nt, Homo sapiens
  source 1..117: mol_type = other RNA
ctcctccacagcccctgctcatccgagaacctcgtttccttcccagaagtcctccttacttctcttcccacagagcccgtgtcgctttcacagccactctccacacacacgcacgtc

SEQ ID NO: 10774 - RNA, 2301 nt, Homo sapiens
  source 1..2301: mol_type = other RNA
ctcctcccctgcctggcccagcacaggcttccgtgtctccaggtggtagtccatgacgtcccatgcatcccagtacaaggggacatcatcaaatagcacaaactggttccccacggcgccctcagcaatggcctccctgccagaggccaccaggaccaaggacgtcaggcgaccagttgggtccagcttcactcggatgatgccattgtccagagtcacggagccatcagtctcttgcactacgaacacaggctgctggggcagcaggggctgcagtgaggtggggggaggaacaggagcatagcccatgctgggcactgtcaccagggctaggctgtgggccccgcccggtttgggcagggccatcacttcgatccgcttccagggcagtgtgttgacgatgaggaggccctcaggacctggctccccagcacacagggctgcggctgcagcgctgagcagtgtattgccatgggaacggatgtcttcataatggcacatggcttcctctgccaccatctggatgcagcttccagtcaccacatcatggaactggttcagaagaaggagcctccagaggtgctgcagctgggctgctgggtataggaactgggcactgcgggccagggccaggctactgagcagctccacgtcgtgcaggatccgctcacattcccggttccccttcttgatctgggcatgggtggtgtatgtgccattgtgcagctccaagaagagctccccaacccacgtgcacagctgctctgagtcactctccagtgctgagaagagctgtcttggagaagatagctgcaccctgggcagcccatccgtattgctcaggcgcttcaggcggtccagcatggtctgggtggggccaccacccccatccccaaagccaaagaggaaggcactgtggttggcccgccccttgtcccggttgttggccacggtcttcagcacctcctccacgctgccctgcatcccataggagtcgccaggtgggaagtggaccagtacacgggagccatccaggccctcccagaaaaatgtatggtgtgggaaggagttcaccaaattccagctcaatttctgggtgagaaagcgcctgatgccacagccgtgcatgatctgggggagctgtgctgagtagccaaaggtgtccggcagccagaactcagagcacatcttcccaaactcctgcagaaagaagttctggccctgcaaaaactgcctcaccatggcctctccactgggcaggttcccatccatctccacccaggtgccccccacaggcacaaactgcccacggcacgcaaactcctggatgcgggagtacaggccagggtagcggctcttcacccattccagctgctgcgcctgggagcaggcaaagatgaactcagggttccgctccatgagctgcagggcggtcacccagctccgggcacatttcctcacagtctctttgaagggccaaagccaggctgtatcaatgtggcagtgccctgtggcatgaatggtgtgttggctttcacccccatgttggccaaagaacctggaggccagggcctgggccactgggaaggtctcgggctgggcagggtcacacacgttcaccatctgattggctgtgtacagggcctggaagctgcgctggttgtccttcccgaggcccttggctatgcccagcagcagctccagatccaccaggagcatgtggacatcccggtggaacacagctagctcagcccggctcagctggaacatcttctcagggtcaggggctgcaatcatgcttcccttcccggcccccaggagcccattgcaggctacttccacatagagagtgaggcttcgggggtctctttcccccagcctgtcagtcaggacatagctggtcttctcaccctctttggttaaaccctggacaggttctccatcacgccacaccagaccttctccatcactttcccagcaaaggtgaacttcctggcccacccatgcctctgggatggtcagctccacccggaaccagcaggtccaccatgtgggtccgaagctgtcgccgacctgcgcggggcggaagtcccgctggactgcctcctggtagggaagtctctccggcgtcaggaagctggagagcacagccacagggcagctggccccaaaaagcctgccgcggaggttacagtcggtaaagtagagcggcgacacgaacttctccacccgctccagcgtggtgcgccagtgcttcaaggccggcgcagccgccatcgccgggctctcgctcctctttcc

SEQ ID NO: 10775 - RNA, 2004 nt, Homo sapiens
  source 1..2004: mol_type = other RNA
ctcctcccctgcctggcccagcacaggcttccgtgtctccaggtggtagtccatgacgtcccatgcatcccagtacaaggggacatcatcaaatagcacaaactggttccccacggcgccctcagcaatggcctccctgccagaggccaccaggaccaaggacgtcaggcgaccagttgggtccagcttcactcggatgatgccattgtccagagtcacggagccatcagtctcttgcactacgaacacaggctgctggggcagcaggggctgcagtgaggtggggggaggaacaggagcatagcccatgctgggcactgtcaccagggctaggctgtgggccccgcccggtttgggcagggccatcacttcgatccgcttccagggcagtgtgttgacgatgaggaggccctcaggacctggctccccagcacacagggctgcggctgcagcgctgagcagtgtattgccatgggaacggatgtcttcataatggcacatggcttcctctgccaccatctggatgcagcttccagtcaccacatcatggaactggttcagaagaaggagcctccagaggtgctgcagctgggctgctgggtataggaactgggcactgcgggccagggccaggctactgagcagctccacgtcgtgcaggatccgctcacattcccggttccccttcttgatctgggcatgggtggtgtatgtgccattgtgcagctccaagaagagctccccaacccacgtgcacagctgctctgagtcactctccagtgctgagaagagctgtcttggagaagatagctgcaccctgggcagcccatccgtattgctcaggcgcttcaggcggtccagcatggtctgggtggggccaccacccccatccccaaagccaaagaggaaggcactgtggttggcccgccccttgtcccggttgttggccacggtcttcagcacctcctccacgctgccctgcatcccataggagtcgccaggtgggaagtggaccagtacacgggagccatccaggccctcccagaaaaatgtatggtgtgggaaggagttcaccaaattccagctcaatttctgggtgagaaagcgcctgatgccacagccgtgcatgatctgggggagctgtgctgagtagccaaaggtgtccggcagccagaactcagagcacatcttcccaaactcctgcagaaagaagttctggccctgcaaaaactgcctcaccatggcctctccactgggcaggttcccatccatctccacccaggtgccccccacaggcacaaactgcccacggcacgcaaactcctggatgcgggagtacaggccagggtagcggctcttcacccattccagctgctgcgccttggctatgcccagcagcagctccagatccaccaggagcatgtggacatcccggtggaacacagctagctcagcccggctcagctggaacatcttctcagggtcaggggctgcaatcatgcttcccttcccggcccccaggagcccattgcaggctacttccacatagagagtgaggcttcgggggtctctttcccccagcctgtcagtcaggacatagctggtcttctcaccctctttggttaaaccctggacaggttctccatcacgccacaccagaccttctccatcactttcccagcaaaggtgaacttcctggcccacccatgcctctgggatggtcagctccacccggaaccagcaggtccaccatgtgggtccgaagctgtcgccgacctgcgcggggcggaagtcccgctggactgcctcctggtagggaagtctctccggcgtcaggaagctggagagcacagccacagggcagctggccccaaaaagcctgccgcggaggttacagtcggtaaagtagagcggcgacacgaacttctccacccgctccagcgtggtgcgccagtgcttcaaggccggcgcagccgccatcgccgggctctcgctcctctttcc

SEQ ID NO: 10776 - RNA, 2352 nt, Homo sapiens
  source 1..2352: mol_type = other RNA
ctcctcccctgcctggcccagcacaggcttccgtgtctccaggtggtagtccatgacgtcccatgcatcccagtacaaggggacatcatcaaatagcacaaactggttccccacggcgccctcagcaatggcctccctgccagaggccaccaggaccaaggacgtcaggcgaccagttgggtccagcttcactcggatgatgccattgtccagagtcacggagccatcagtctttgtgggaggaggccttgaggctgagtctgtaggggctcttgcactacgaacacaggctgctggggcagcaggggctgcagtgaggtggggggaggaacaggagcatagcccatgctgggcactgtcaccagggctgggggtgaggcctaggctgtgggccccgcccggtttgggcagggccatcacttcgatccgcttccagggcagtgtgttgacgatgaggaggccctcaggacctggctccccagcacacagggctgcggctgcagcgctgagcagtgtattgccatgggaacggatgtcttcataatggcacatggcttcctctgccaccatctggatgcagcttccagtcaccacatcatggaactggttcagaagaaggagcctccagaggtgctgcagctgggctgctgggtataggaactgggcactgcgggccagggccaggctactgagcagctccacgtcgtgcaggatccgctcacattcccggttccccttcttgatctgggcatgggtggtgtatgtgccattgtgcagctccaagaagagctccccaacccacgtgcacagctgctctgagtcactctccagtgctgagaagagctgtcttggagaagatagctgcaccctgggcagcccatccgtattgctcaggcgcttcaggcggtccagcatggtctgggtggggccaccacccccatccccaaagccaaagaggaaggcactgtggttggcccgccccttgtcccggttgttggccacggtcttcagcacctcctccacgctgccctgcatcccataggagtcgccaggtgggaagtggaccagtacacgggagccatccaggccctcccagaaaaatgtatggtgtgggaaggagttcaccaaattccagctcaatttctgggtgagaaagcgcctgatgccacagccgtgcatgatctgggggagctgtgctgagtagccaaaggtgtccggcagccagaactcagagcacatcttcccaaactcctgcagaaagaagttctggccctgcaaaaactgcctcaccatggcctctccactgggcaggttcccatccatctccacccaggtgccccccacaggcacaaactgcccacggcacgcaaactcctggatgcgggagtacaggccagggtagcggctcttcacccattccagctgctgcgcctgggagcaggcaaagatgaactcagggttccgctccatgagctgcagggcggtcacccagctccgggcacatttcctcacagtctctttgaagggccaaagccaggctgtatcaatgtggcagtgccctgtggcatgaatggtgtgttggctttcacccccatgttggccaaagaacctggaggccagggcctgggccactgggaaggtctcgggctgggcagggtcacacacgttcaccatctgattggctgtgtacagggcctggaagctgcgctggttgtccttcccgaggcccttggctatgcccagcagcagctccagatccaccaggagcatgtggacatcccggtggaacacagctagctcagcccggctcagctggaacatcttctcagggtcaggggctgcaatcatgcttcccttcccggcccccaggagcccattgcaggctacttccacatagagagtgaggcttcgggggtctctttcccccagcctgtcagtcaggacatagctggtcttctcaccctctttggttaaaccctggacaggttctccatcacgccacaccagaccttctccatcactttcccagcaaaggtgaacttcctggcccacccatgcctctgggatggtcagctccacccggaaccagcaggtccaccatgtgggtccgaagctgtcgccgacctgcgcggggcggaagtcccgctggactgcctcctggtagggaagtctctccggcgtcaggaagctggagagcacagccacagggcagctggccccaaaaagcctgccgcggaggttacagtcggtaaagtagagcggcgacacgaacttctccacccgctccagcgtggtgcgccagtgcttcaaggccggcgcagccgccatcgccgggctctcgctcctctttcc

SEQ ID NO: 10777 - RNA, 956 nt, Homo sapiens
  source 1..956: mol_type = other RNA
ctcctcccctgcctggcccagcggttttggtcctgtggacccagcagcctggcgtctgacttagcaattctgtgtcactgctgcttccaccggctgcagaatcggggctttcaggaacgtctccagccagctcctgagtctttccgggccccccactcatgacccgggtgaacctaacgtgcgttcacctcccatttatgtgagggtgacgttctaacaacttgagaccacgaccatgcccaggggagtgtgggctctctgcaggcatccggcgcgtttccagacacagctgaggccggacgtgctgggtcagtgagggctgagatgtgcagcctcgggcctttcctgggacactcccccgaccctgcctgtcatcccgacatgcccctcagcattcctacactcataggaatgagtcctgcactcataggaaatggggggctcaggcaggtgggtggtctgtcctcaggacaacccaaatccccgacccaaacctcttcactcccgtctcgtgctcaccaccgtgcagcctcttaatgaaccacctcccacccctcggagccaggcagggcgcgctgtgcatggggatgggtctgagctggtcttgagtcggtggaaccctggaagaagtggctccgtcattctcgttgccatgggccatctggccctgcaggtgtggatcggggacagtgaggatgcaggactggtctgcagctgcagagtccaaagacgggagcccaaagtccccatcttcaaagactatcactttgcaggtagagttccagtggattaatctgggggcacacaaacatttggtccataaaagactatcactttgcaggtacagttccagtagattaatctgggggcacacaaacatttggtccacaatagggcccatggtgggggggggacctgggcaccaccgagggtggaagcaagttgtggaatgtgga

SEQ ID NO: 10778 - RNA, 49 nt, Homo sapiens
  source 1..49: mol_type = other RNA
ctcctcccctgcctggcccagctgcctccttcggagcctgctcaggaat

SEQ ID NO: 10779 - RNA, 2207 nt, Homo sapiens
  source 1..2207: mol_type = other RNA
ctcctctgttttctttcctagaatgtatggtcacccaagctctgctgtccccctgggtttcagttatttatcactagccagcagctctggcatattcatggcagctggtactcggccttctaattggacccttccctcttccacctgtttttggggactacactttgcaaaggagagtggcaaccatccatgtggcaagccccaagccccctttcctgactacttaactttgaggatgtaaacacagaggtcaggtgactcgggggagtcatggtcacttggcgagggggcttggatttgaacctgggcatttaccttcagaatctgagtttgtatctatggtgctctagtgcctctaccctagttctaaatgccctgtgtttagaatgtgttcaggctgctctgatcagattaagagcactgctgaacacacttttccttcaatgcttttcactgctgtagggctcttacctactcccctggagaggaccacctaggttgtctccactgctaggcttcccaaaccccatgctgatgagtatcctcatacacaggacctccagggaaacaccccaggtgcacaggctcagagcagcaggttgcaggatattcctataattaacttctccaagcacaaagtgtgctccttctgtgaattcctgaagccgtgcaggctcctacttctaagctacacaactgcaaaccaaaaggtgcttcgaggagctgtcatcgtgaagtgaccggctgacgggactgtgtactggaaaggaatctgcaaacggtttcatgctggacaaatgtgtgggccactcacattgttgctgaacagcaggatctgtctttagggtgaagtgtgggcaatttccattgaggggatgtacctgccaccgtctggtttgtggaggagagagtgcccctggaatccaacccacaggcaggagcctaggaccaaaatcaagcaagctcttctggcctgttagtatgcaggtcgagggaggggccttgattcacaatggctcagtgctctcaccaccgggccctaatgcacaggctgaggcaagggcagcagggctcggattcttaaatccttgtggactctgagcacacaatccactctccacaagcaagcatagtggacttcctcaggtagaaagcagcccagcaatttactccttggcacacagctccaaagatgatccccaacaatgctacccctacccccagcatatgccacccattcctgcccaagatggaaaaattactaggctggcctgtaaatgctccggtcaatacagtgacagtctgggacatctgaatcctggtcttaagaaggctgaacgcttctaattccctcctcttggaatccagcctctgtattgttagaagcctgagccacagggcaaggatacagagaggtgagctgaggagctctggacagaagtccagtggagctcccaacagcagccagcaccactgatggccacgtgagcaagaaaccttgcacgttcagcccagttgagcctctgaatgactgcagccccagtaccatcacatggaacagaagaactgcccaactgagcccatcccatgcaccaaatccttaaaatgtaaatccgatgttttctggttatctacgactgcataacaaatcatgccaaaatgcagtggctttaaacagcagtctttcattacttcttgcagttcctgtaggtcagaaattcgagaggagcagggctgggcggctgtggctcaggatctctcatgcgctcagtcctcatggagggctaggttggggtcagttgtgccaaactgagtaaaccactcaccctctctggtcttcagtttctcacttggtttttcagatgtaaatcccatctacatgtatttcacttggtatcttcggaagacacgggcagagctggttttgacagtgatgcagttgctggcaaatccgtttgcatccaacattgtcttgaaatttgggtcacctcttcacaaatcctgggtctgtgcgcgccgcgatgcgccggggctcctgcgctgtcctgcgctccgctctcggcaccacctttcgtggctccaccgcccccagcccgcacccgagcgctgaggtggcaagggcaggtctgcgtgcgagccccctgcgggctggcagccaggtgcgcgagggccgcccttgccggcgctcccagcccgcgctgtctgct

SEQ ID NO: 10780 - RNA, 5186 nt, Homo sapiens
  source 1..5186: mol_type = other RNA
ctcctgactccaggtcctgtgtctaccagccgtcccgggggtcctgggggacccggctccccacggtcacccttgggtccagatgatccagggctgccatttcgtccatcctctccaggatctccctggtctcccttttcacccacaggcccccgaactccaggtgccccccgaaggccacgctcgcctgcttttccaggcaaacccgggtcacccggaggaccctcgtcacctttctctccaacttcaccatctcgtcctcgggggccaacaggtcctggggggccaggccgcccagggtctcccttctctccaggaggccctgagtcacctgggggtcctgctctgccagtaaggccaatgggaccccggtctccagggtctcccttggggccagggtctccaggaagaaccaagccgggtgggccccgttccccttggactccggtagctcctctgggcccagcgggccccacatctcccttttctcctttgggtccagcaacagcaggtcccaccactgcagggtccccagggcgaccaggctcccccttctctccttggcggccagtgggtcctggtggcccttcaggacccttggctccaggacgtccagcaacccctggcagcccccgggatcccgctgggcctgggggtccacgttcgcccttctctccagcctcacccaggggccctggaaagccccggtcacctttggggccaatagctccaggaggtccccgtgggccctgctcacccggagacccaggttgtcctgggaggcctggagctccatcctcagagtcacctttttctcctttctttccaggggggccaacggggccttggggtccagggcttccgggaagacccggcagcccaggctccccaggagcaatgccaccttcacctggtccagggggaccccgctccccacgatcgcctttgtcacccttcatggctgttccaggaagccctggggggccacggggtcctgggtcccccagtggtccacgaggtccaggggggcccgatggtccagggtcccctttccgcccaggaagcccaggtccttcacctccgatgacttgtccgggagcccccggctccccctttgggcctcgaggtcctcgctctcccgggtccccacgagggccaggcaaccctggagagccctttaggccaggggctccaggggtcccaggattcccggcgcggccagggctgcctggacgcccatctgctccagggaagcccctctcgcccttggcagtggcacttccagggggcccctgggggccgggagcaccggtcctgcccgggaggccagggtcgccaggaggcccaacttgtcctctcaggcccatctctccaggttcccccttctggccctttggacaatacactgggcagggctctggccggggctgagtagtgaaggatgcctgacacagggctgtggccagaccactgactgcctggtccaggcttggcccatcatccacggcgaagaaggtctggacagagtccatacccggcgccaagcgacgcagctgctctgggtccgctccagccattcccaacatcaccacattaagcccagaagcctgggcctcacggatggggctgaatatgtcacctctcaagggttcatccactagcagaaccatcacccctggtacgtgctggcggcgcccaggagcatctggtgccaacatgtatctgtgagctgtgaccacggctgtgcccaggttgttcccacttgggtccatgtagggcatgtcacggatcctttgcaagataatgccaaggtcatgggagccattcagtgggaacagtggggagggccgatgactgtaagacagcaggccaacctgaactgcctgtggcccaagaggcccaagtgccaacaccagacgctccaggaccctcctcgtagcctccgcacggtgagcattgtcttgagtggcatgtggtaggaacaccacatccgccaggccacgggggcacactggcgtctgtgtgacagatgcctcaggaccccgcacaccatccaggacaggcgtcagggagaagatgtaagagacgccaggctctagccctgtcacccgctgggagcttgagatccctggaagtgtctgcggggacccaggcacttcctggccagggcctctgagtggccgccaggataggatgtagctggatgccctggacactggagtccaggccaaagtcaccgagtcgatcgaggtgtccaccacacgtagttcaatgcttggaacacgaggtgactcagtgcgcgcagtcacctctgcagagggcccttctccagctggccctaggacactcagcctcacgcggtactgtgtcgctggctccagcccgtccaggtgatagctgctgagctcgggccccaggacccgggactgttcctggccaccctcaggttgccagtgcagaaggaagccctgcgctctgggcaccggctcccagcgcagcctcagcgagtgctccccgcgctgcaccacgtgaagcgtccccagggctggcggagcctcaggcggcgtagtgacaacaatggagacaggtgtgccctcgcggtccccgacaagtgcagtcactcgcactgagtagctgactccaccttcgagaccccggatctctgcagagtctgtgtttcctgggagtatctggtgcctcatggggccgccttcactccggccccaggccagtctgtaagctgtggctccagtgacccctacccaggtgatccgtagaacgtcgctggaagcattgaggatctgcagcctcgacacacgacccacaggctcaggggcagtcctcacaaccacagaggcagggggcccatccacgccagccacatgggccctcacatgcaccgtatactcagtatctggctccagtccatccagctcagccaccgtggcctccccagaaaccaactgggatttctctgggccgtgggctgagtgccaggaaaccctgtatcctgtggcgccaggaaccctggtccaggtaatggtgacagatgagctgctggcctgagtcacatggaccgtcctcactgggcccagtgggtccgttcgagccacgatgactgcagcagggccctcctctctgcctcgcagtaccgacacagccacctggtaggtggttccaggctgcagccctgtgatgtctgtggcagtagagtctgggggcagtgtctggctggactccggaccactgcctgtgctccagctaatccgaaatccactggctccagggacgggtccccaggccaccctcactcgcgttgcatctgacaccacaacccgcagccctggaacagcaagtggagtttccggctcccggcggacagtgaggacactggcactgccctcacggggacccactcgagcagacacccgcacagtgtagctaagcccagcctgaacgtcatccaagtcgaatgctgtctgactcccaggaagcaccagggtccgctcaaccccctgggtgctgcgcacaatgatgcggtactgggtggcaccagggactgggctccaggacactcgcacccgctgcccgggcagctcggtggcttgcaggtctgttacagggctcacaggcagctctggtccagtgggaaccacggttgcaggggtggccacctcgtggccctccagcagagtgtagagtgtgaggcggtactcagtgcccggctgcagcccatccaactggtagcgggtcacatcagagggcagtaccaccttctgcggtggctccaagccagtctcacgccgccattccaaccggtagccacgggcctcaggcaccaagttccaggaaaggaggatggatgtggggcccaggatgaccgggcgcagggtctgctcaacagaagcgtcagtgcgagccatcagggaagtggcgggccccacactgcggccaaatagggtgctcacggtcacctcatagtccgtgccaggctccaagtcacgcagcaacactgaaccctgcccagggcccagctcctgctgctgtgtgggcccaccactgaggacccgccatgtcacacggtagccagtggcacctggcacactccgccaggccaccaggaggctgtgggctgtggtattctggatggtcagttccggcccttctagggcagtggtccgagctgtcccgctcacagcctccccgatgctgttggcgtagagggcaatcacagtcacttggtactcggtcagtggccggagaccccgcagccgcacactggtctcaccagctgggacgttcacctcctgccgctcactcggcagtggctgtcccagccccgtcagaggagtgtactggaccttgtagccagtcacagggccactggccgctgtccactgtactctcaaggattggctgcttggctcagacagcaccaggtctcgtggagcagaggtcgagtcatccggaggtcgggtcacaggcacgccaccagcagtcgtgcacactctccgggaaacgaggggcagtagtgtcctcaagatgctgaagtcattgacgaagaagaagaagtcactggtgggctgtgaggcaactcgcttcagctcctcagggtcagcattcttgatccccacagcaaatagcttgaccccctgccccttcagcctttgggcagctgtgtccaccaggtcctgggacttcccgtctgtgatcaggatgcagaccttggggacaccaggtcgggccagctggggcaggaagacatggtcagccacatggagaattgcagcccctgtgcgagtgttgccccccttgtagctaagctcacggatggcgcggatcacatcacccccagagccaagtgcatccaggccgaactctgtccgtgggtcatcgctgtactgcactgtggcaaagcgcacaccctgtgcactggctgctccagagaaaggcagcaccagcccttcgagaaagctgcggacctcgcggaaattgctgcggccaatggatgaggagccatccagtaagaacacaatgtcagcggcgtaaaggcgcgtgcaggtcactctctccctgtgctgggctcgcactcggggcgcctctgccaggatcccggcgcagagcgcggccaccagaagccgcagcgtcatcctgcgcgtccgcccgctcccgccgccgccgctgca

SEQ ID NO: 10781 - RNA, 5213 nt, Homo sapiens
  source 1..5213: mol_type = other RNA
ctcctgactccaggtcctgtgtctaccagccgtcccgggggtcctgggggacccggctccccacggtcacccttgggtccagatgatccagggctgccatttcgtccatcctctccaggatctccctggtctcccttttcacccacaggcccccgaactccaggtgccccccgaaggccacgctcgcctgcttttccaggcaaacccgggtcacccggaggaccctcgtcacctttctctccaacttcaccatctcgtcctcgggggccaacaggtcctggggggccaggccgcccagggtctcccttctctccaggaggccctgagtcacctgggggtcctgctctgccagtaaggccaatgggaccccggtctccagggtctcccttggggccagggtctccaggaagaaccaagccgggtgggccccgttccccttggactccggtagctcctctgggcccagcgggccccacatctcccttttctcctttgggtccagcaacagcaggtcccaccactgcagggtccccagggcgaccaggctcccccttctctccttggcggccagtgggtcctggtggcccttcaggacccttggctccaggacgtccagcaacccctggcagcccccgggatcccgctgggcctgggggtccacgttcgcccttctctccagcctcacccaggggccctggaaagccccggtcacctttggggccaatagctccaggaggtccccgtgggccctgctcacccggagacccaggttgtcctgggaggcctggagctccatcctcagagtcacctttttctcctttctttccaggggggccaacggggccttggggtccagggcttccgggaagacccggcagcccaggctccccaggagcaatgccaccttcacctggtccagggggaccccgctccccacgatcgcctttgtcacccttcatggctgttccaggaagccctggggggccacggggtcctgggtcccccagtggtccacgaggtccaggggggcccgatggtccagggtcccctttccgcccaggaagcccaggtccttcacctccgatgacttgtccgggagcccccggctccccctttgggcctcgaggtcctcgctctcccgggtccccacgagggccaggcaaccctggagagccctttaggccaggggctccaggggtcccaggattcccggcgcggccagggctgcctggacgcccatctgctccagggaagcccctctcgcccttggcagtggcacttccagggggcccctgggggccgggagcaccggtcctgcccgggaggccagggtcgccaggaggcccaacttgtcctctcaggcccatctctccaggttcccccttctggccctttggacaatacactgggcagggctctggccggggctgagtagtgaaggatgcctgacacagggctgtggccagaccactgactgcctggtccaggcttggcccatcatccacggcgaagaaggtctggacagagtccatacccggcgccaagcgacgcagctgctctgggtccgctccagccattcccaacatcaccacattaagcccagaagcctgggcctcacggatggggctgaatatgtcacctctcaagggttcatccactagcagaaccatcacccctggtacgtgctggcggcgcccaggagcatctggtgccaacatgtatctgtgagctgtgaccacggctgtgcccaggttgttcccacttgggtccatgtagggcatgtcacggatcctttgcaagataatgccaaggtcatgggagccattcagtgggaacagtggggagggccgatgactgtaagacagcaggccaacctgaactgcctgtggcccaagaggcccaagtgccaacaccagacgctccaggaccctcctcgtagcctccgcacggtgagcattgtcttgagtggcatgtggtaggaacaccacatccgccaggccacgggggcacactggcgtctgtgtgacagatgcctcaggaccccgcacaccatccaggacaggcgtcagggagaagatgtaagagacgccaggctctagccctgtcacccgctgggagcttgagatccctggaagtgtctgcggggacccaggcacttcctggccagggcctctgagtggccgccaggataggatgtagctggatgccctggacactggagtccaggccaaagtcaccgagtcgatcgaggtgtccaccacacgtagttcaatgcttggaacacgaggtgactcagtgcgcgcagtcacctctgcagagggcccttctccagctggccctaggacactcagcctcacgcggtactgtgtcgctggctccagcccgtccaggtgatagctgctgagctcgggccccaggacccgggactgttcctggccaccctcaggttgccagtgcagaaggaagccctgcgctctgggcaccggctcccagcgcagcctcagcgagtgctccccgcgctgcaccacgtgaagcgtccccagggctggcggagcctcaggcggcgtagtgacaacaatggagacaggtgtgccctcgcggtccccgacaagtgcagtcactcgcactgagtagctgactccaccttcgagaccccggatctctgcagagtctgtgtttcctgggagtatctggtgcctcatggggccgccttcactccggccccaggccagtctgtaagctgtggctccagtgacccctacccaggtgatccgtagaacgtcgctggaagcattgaggatctgcagcctcgacacacgacccacaggctcaggggcagtcctcacaaccacagaggcagggggcccatccacgccagccacatgggccctcacatgcaccgtatactcagtatctggctccagtccatccagctcagccaccgtggcctccccagaaaccaactgggatttctctgggccgtgggctgagtgccaggaaaccctgtatcctgtggcgccaggaaccctggtccaggtaatggtgacagatgagctgctggcctgagtcacatggaccgtcctcactgggcccagtgggtccgttcgagccacgatgactgcagcagggccctcctctctgcctcgcagtaccgacacagccacctggtaggtggttccaggctgcagccctgtgatgtctgtggcagtagagtctgggggcagtgtctggctggactccggaccactgcctgtgctccagctaatccgaaatccactggctccagggacgggtccccaggccaccctcactcgcgttgcatctgacaccacaacccgcagccctggaacagcaagtggagtttccggctcccggcggacagtgaggacactggcactgccctcacggggacccactcgagcagacacccgcacagtgtagctaagcccagcctgaacgtcatccaagtcgaatgctgtctgactcccaggaagcaccagggtccgctcaaccccctgggtgctgcgcacaatgatgcggtactgggtggcaccagggactgggctccaggacactcgcacccgctgcccgggcagctcggtggcttgcaggtctgttacagggctcacaggcagctctggtccagtgggaaccacggttgcaggggtggccacctcgtggccctccagcagagtgtagagtgtgaggcggtactcagtgcccggctgcagcccatccaactggtagcgggtcacatcagagggcagtaccaccttctgcggtggctccaagccagtctcacgccgccattccaaccggtagccacgggcctcaggcaccaagttccaggaaaggaggatggatgtggggcccaggatgaccgggcgcagggtctgctcaacagaagcgtcagtgcgagccatcagggaagtggcgggccccacactgcggccaaatagggtgctcacggtcacctcatagtccgtgccaggctccaagtcacgcagcaacactgaaccctgcccagggcccagctcctgctgctgtgtgggcccaccactgaggacccgccatgtcacacggtagccagtggcacctggcacactccgccaggccaccaggaggctgtgggctgtggtattctggatggtcagttccggcccttctagggcagtggtccgagctgtcccgctcacagcctccccgatgctgttggcgtagagggcaatcacagtcacttggtactcggtcagtggccggagaccccgcagccgcacactggtctcaccagctgggacgttcacctcctgccgctcactcggcagtggctgtcccagccccgtcagaggagtgtactggaccttgtagccagtcacagggccactggccgctgtccactgtactctcaaggattggctgcttggctcagacagcaccaggtctcgtggagcagaggtcgagtcatccggaggtcgggtcacaggcacgccaccagcagtcgtgcacactctccgggaaacgaggggcagtagtgtcctcaagatgctgaagtcattgacgaagaagaagaagtcactggtgggctgtgaggcaactcgcttcagctcctcagggtcagcattcttgatccccacagcaaatagcttgaccccctgccccttcagcctttgggcagctgtgtccaccaggtcctgggacttcccgtctgtgatcaggatgcagaccttggggacaccaggtcgggccagctggggcaggaagacatggtcagccacatggagaattgcagcccctgtgcgagtgttgccccccttgtagctaagctcacggatggcgcggatcacatcacccccagagccaagtgcatccaggccgaactctgtccgtgggtcatcgctgtactgcactgtggcaaagcgcacaccctgtgcactggctgctccagagaaaggcagcaccagcccttcgagaaagctgcggacctcgcggaaattgctgcggccaatggatgaggagccatccagtaagaacacaatgtcagcggcgtaaaggcgcgtgcaggtcactctctccctgtgctgggctcgcactcggggcgcctctgccaggatcccggcgcagagcgcggccaccagaagccgcagcgtcatcctgcgcgtccgcccgctcccgccgccgccgctgcagtctctcgggcagagcagagaaaagtc

SEQ ID NO: 10782 - RNA, 6900 nt, Homo sapiens
  source 1..6900: mol_type = other RNA
ctcctgactccaggtcctgtgtgccaacagggagggtgaaaacagtcacaagggccctgacactttcacagctggcacagcctccaggccactcctcctgcggcctcaggacaatgccatgaccagcccatttcgcagatcaggaaaccgaggcagcacacagcaggagcatcagagtctggccacacagctttgcttctcagctccgccagggtagccaggtgaccaggacgatcccttcacctctctgaacctgaggctttcccctgtaatatggaagcaataaacttccctccccgtattagttttctattgctgcataacacaaaaccataagcttactggcttcaaataacacccacttattagctcctagttccgtaagtcagaagtcaggacatggcaggactgggtcctctgcttggggtctcaaaggctgaaatcggtgtgtcagcccaggtgccttctcatctgctcggggtccgaaaggctgaaatcagtgtagcagtggggtgccttctcatcttccctcaaggggaaactctacttccgtgctcactcagggtgttagcaagagtcagatccctgcagctatggcactaagatccctatctctctgttgaccatcagcaggggccactctcagctcctagaggtcactcacattcccttccacatagtcccctccatcttcaaaccagcatcccccgcttccatcctgtgcttccagtctcaatctccaggaagaattttgtcccctttagggcttccctgattagggcagggccaccaaggcttatactttcttaaagtctcctgtgcatataagatagcctaggcatgcaggcgaaacctgtcacagtcactggttcctgccacactcaggggagggggctatacaggatatgggtcatggagggtcttcatatagcaattctcccttccacatttgctcacagtaggaaaagcacacaggaggtagtgagcatccacccctgccagcatccctgctccactgtgccaggaaaagaacctttgcccacggaatccacgtccaactcccattttccagcttctcatgtataaagaagaaaacacagtccatcctagggcaccccaggcaatctctccgagtatcctgcactgccccagactctctctaaacagttccaggctctcagccctgctcagggtgagacagcacctctcaggctctcggccctgctcagggtgagacagcacctctcaggctctcggccctgctcagggtgagacagcacctcttgcacagccttcagggctcctgcatgaggatcctgggaggagcctttggctgcaccatggggtgcccagacaccacgtaggtgcctcatggcacatacccttcccttccctctcctgcccttcccttccaagctgagattgagcctcctctcctgcacagatcttcctccgggcaatgtagtcccagccccttttctgaatgagctctgcaaaccccagcccaggccccaccatctgtggctgccacaccctcttccctggtctcactctgctgccttcctgggacccatttccacccggggtggccagccagagtgacggcttggaaatgtgcccgatcacactgtctcttggtctctgtcacacacactcacgcacacacacactcacatccctctcttcagacatcccatggttccctcatggcagacaagctcctccccagtccaggaggccccaaccgtctggctcccagctcccctgcagccccatcccgccatactcctgcttctctcttgcctctggctccagccgaagctgcccccaccacctggcctttgcactgccaatctctcggcctagcatacctttccctttcctgctgggctagttaattcgaagccaccttttggctctaactcaagtgccctcccctggacccttccctcagatccccagatatgccaacccctccacaagcccgcagggctccagggcagcctccccacagctggatggggcattcgcctatgagctgatgtgatccaagcccatcactcaccagacgatctaccacgaggatgaggcaacaggtcggtttgctgcgctattccccaagcccagcctcacccctgacattatcataggcactaaatttgctggaagggaaggagaaagaagaaggacagagggagggatggaaggagggacgaagggagaaatgacacgtgccgtgagctatgcctcttttttctactcagactctcaattgtggacagaagccgcttaattctccttccacacctagcacaggcacccagaatgtcagccccacgaaatgttagctgagcccctgggtgctaaagtgaacaacttccacctcctccttgctaaagatttcaccaggcaagatgcaaacatcagttcaacaaaacagaaaaaaaaaaatgactggaatccctcttttcctataagaaaatagctgctctacactaatatcctctggaataaattgttattagttaattttttaacaccacacagagaccaatcattaacaaatgtgtgggctcactttcagtgatgtatattcctgagaactcacactcgggctcctgcccactggcttgctcatttgctccaggaatttccaacagggtgagactatttaacctgaagccatcatggaactctttgtttattgttgttttttttgggtttttctccctcgattttaatttttttatgggaacatgggaataggtatgaggaggggtgctagacgtcactatcacgtacccaagagtcaatcaatatttaccatgcacctactatgagcatagctctattctacagaccaggatggagctggaacaacacaaatccctaaagaaaaaggatgcaaatatactccccaagtagaaaagggctggaaaaatattacaggaaaataatcacattaaaatgtcaacactgtttgaagtaatgatcttaaggaaaaggcaggctgtattagactcccaacggggaagcgagcggggaaagccagcccaggtgaatgagagtgcaggcaacgctctgagcttaccccacatggcatggtattaaatgtgctccaaaactcacccttcccattaaaaaaaaatgagctaaattataaattctccctaaatcttttgttatttcacatcaaagcagaaccagctacttgcaaggattaggggaaagaactaaccaaagcaaacagctagtgctcccttagctcagtgtctacatgcagtttccttcctgagcccagaggcaaccctaaggaacccaggggctggtggtcagctcagcgcagccacagcctcacgtcccagctggaatgagactcagcctctgaccctgggtcttttacccaactcagtattctgactgcctcaagccagctcccccactaggaaatcagggggcaacgccttgagcggagcttcccggtgcatgccagcagtctcctgaaccagctccagggcagtacagggtgaagggaggaagttctagagggatgcctgatttcacccagcagctcagaccaggaaagccctccctcctgcatcttgaggcccaaaggaagacaagggcatctgggagcctcaaaactgcaccagatcagaacctcctgctcttatccaccaagacatggcctttggtgaaaacttctccacagtgataggaggaggcgaatgctagctcatggtgaccaggatcttcctgtgtcccaggaactgtgctaaacgctttacagaattcatctcatctcagcatcataactgctcgtctaagggggtattaatataagtaaagtaatcctcattctgcagatgggaaaactgtggatcagagatgttaggtagatcttccaaagccacacagtgaacccaggcagtctgacaccagagaccacacatctgcaagcaccccacagaccttgtctgttggcatccaatgtcaaggcatcaccttatcagaggtggcaggagattccaaggtgattctgactccaggagcccacagactacatagggaaataagcctaatgtgtggattacaagactggccccaattctccacctctcctgtatctacatatgactttcctgctcccccaaccaaaggggtcaagtgtatttccctctctttgacctgaagttggccaataggctaacagaatcagcataagtgaaggtttccagcctaggccctaagaggtcccatgtatcttcaccactacacaagactaacatggctggtttagactgcaggtccaagaaggataagagatgcacggagaagagccagcctggaccttcgaccctgccaaccttcagaaacccaaggactgaaagctcaatgctgtagggccacggaggtctggagaatgcttttgcagaagcctgtgatacctggcagagaatgaatgggatacagcacagaaggggacaagtttgagaggcctggcacttattacatatgtgccctgtcattttacttgtcaaaatgttatgcccctagccagaccatgagcttcccggatgcacgatgcccctttgcataccctcacaccatgctccatgcacactgtagtgcttaatgcgtcagcaaataggtaagtaatcatggccgggccacaagaccaagatgaaaatttataacagcatttccccatttcactgaaacctgtacaccagctttgtggtttttggcatgcctgtgtcttccaagcactaccttcatggtttcttcgcatatttctgtgtattaccaccactacattattactattttcaagtcatgttcttttttatgtaaataagcttgattggaaagaacacttctataggccccctcttgatggaaaacctgtatctctggttgtatatagagaataacaggaaaataaagaatgtggggtaggggccaggcagatccccgaaaaacaggtgacaagacagtcctgacaccgtggaggtcatcagatctcagaagctttgcacaaaaaacccggccaataaacgtgccaaagtcagcaaccatttgactcacgtgactcaagaaacgcagagtcaccccaggagtaacgctgcctaagacaatgccttcctgccaaagggaagcagaaagatcatttttggcatatcttcctgacttcattgaaactccagagctagtgattacaataaggcaacaattttttctatatatggatacaaactttcaagagataattgaaccaaaaagtaatgccataacaatacaactcattaggaagagtattgcaagaccaatggtgactttttaaaagggttgtattacaaacaggagcatagtatgtataataaacacacttcttaggtcgtatagccacagctcccgtcttctcagtgcagggctgatccatttcgtggctgccaactaatcaacgtcaaagtctacagatgtcgtgaccattagataaggtgcgttgccaagctacccatccaaccgacttgctttaacaaacaggaacacgagtcccagcccattaaagacgggaccttcaacaactctacagacagctgattctctgccatcgccttgcctgactttcaatacataaatcttgtcccagtggccattctggttaaatgaactgggaaatgaaagagtacatctgcctctgtgtgcttttgtgactacaggtatgtatacgtctgtcagctagatggctggagccaggaatgggggtgaaacacacatatctattccatgtaaaggacagaggaccgctttccagtaagttgcaggatgagggaggcagaagctgggtggtgcagatagggatgggccaggcctcagactcacttggattcaagatcctctttaagcttcccctttatataaatgtgaccatgggccggttactcagcctcgctagctttctggccctacctcaagggtttagaggactattcaataaaaggaagtatgatggctccttttataacaagagttgacaataagcacattttcactccagccgttgatcgctgaccagatgattggctctgtgaggaacagtgaccctgcctatcttgttccctggatattgttaaataaaatttgaatggacataatgtttaggcttggatcacatatcttagtccaacctttaatttcttagtaatggcacaaaacataaaaactgcttcagtcttcccatgagattctttctatctgaggtttgaaagggcaactacaggccacatgcagctcccagacatgttttgttttgatcacattgtgcttttataaagttgatatggcagagactgtagttcactacctgatagtcattctcaccctccccttccgcggaacctgctcttgttagagtagcaatacacctatcttaagcaaacaaacaaacaaacaaaaagaaaaagctacacttcccaggctccctggcagctgggagtagccttttgatgtcctaagaccaaggaggtataagtgggtgtcactgggcagtgctcccaagaaggcaatgtcaaactcggcaggtggacacccctgtgcctctccctaccctctttgtcctgcctagaaaatgtacttgttgctggaggtgaagcaaccatgttgcaaccagaattcagtatgaaattcactgaacgtcccaccctacgacagggacgccatcatgctgtctggacttctggtggaaggaaaacctttatcttctttaagccagtgttatttaggttttctattacataaagtcaacccaatccctaatagataaacttgtcaatatttaaaaatcatatccgatagggtttgaatatttgtcccctccaaatctcatgttgaaatgga

SEQ ID NO: 10783 - RNA, 612 nt, Homo sapiens
  source 1..612: mol_type = other RNA
ctcggccgcggcgcgtagcccccgccacatcgggcctggctctcctcagccgccggctcggctcggtgcgcgcgggggtcttgagctcaccgccggcggggcggggttacatggcgcgcgaggaggggggagagaagaggagagcctaggtgccctcctctcccctcccccccggcggcggcgcgcgcacggccctcgccggcctcacccctccgcaccccgcccgcctgctcttcaccggccaggccctgccgggtcgccgcggcctcggcgccccaccccctcccgggccagcggggggctgggagggggcgaggaggaagggggttctcctctcccctccccggagggggccgcagcggcggctccggctcctcctctccctcacaccccctcccgcccccctctacctgcgggggacacgggcagaaggaggcggtgcacggacggggcccggcgacaactgtcagttagaagccccgctgggcggtgaggggggagaaaggggaggggcagggagagaagggggagggcactcagccccccggctgggaagagctgtggagagaagcaaagaaagaggccctgtcgccatccccggtgcgcatgcgt

SEQ ID NO: 10784 - RNA, 618 nt, Homo sapiens
  source 1..618: mol_type = other RNA
ctcggccgcggcgcgtagcccccgccacatcgggcctggctctcctcagccgccggctcggctcggtgcgcgcgggggtcttgagctcaccgccggcggggcggggttacatggcgcgcgaggaggggggagagaagaggagagcctaggtgccctcctctcccctcccccccggcggcggcgcgcgcacggccctcgccggcctcacccctccgcaccccgcccgcctgctcttcaccggccaggccctgccgggtcgccgcggcctcggcgccccaccccctcccgggccagcggggggctgggagggggcgaggaggaagggggttctcctctcccctccccggagggggccgcagcggcggctccggctcctcctctccctcacaccccctcccgcccccctctacctgcgggggacacgggcagaaggaggcggtgcacggacggggcccggcgacaactgtcagttagaagccccgctgggcggtgaggggggagaaaggggaggggcagggagagaagggggagggcactcagccccccggctgggaagagctgtggagagaagcaaagaaagaggccctgtcgccatccccggtgcgcatgcgtagtaga

SEQ ID NO: 10785 - RNA, 619 nt, Homo sapiens
  source 1..619: mol_type = other RNA
ctcggccgcggcgcgtagcccccgccacatcgggcctggctctcctcagccgccggctcggctcggtgcgcgcgggggtcttgagctcaccgccggcggggcggggttacatggcgcgcgaggaggggggagagaagaggagagcctaggtgccctcctctcccctcccccccggcggcggcgcgcgcacggccctcgccggcctcacccctccgcaccccgcccgcctgctcttcaccggccaggccctgccgggtcgccgcggcctcggcgccccaccccctcccgggccagcggggggctgggagggggcgaggaggaagggggttctcctctcccctccccggagggggccgcagcggcggctccggctcctcctctccctcacaccccctcccgcccccctctacctgcgggggacacgggcagaaggaggcggtgcacggacggggcccggcgacaactgtcagttagaagccccgctgggcggtgaggggggagaaaggggaggggcagggagagaagggggagggcactcagccccccggctgggaagagctgtggagagaagcaaagaaagaggccctgtcgccatccccggtgcgcatgcgtagtagaa

SEQ ID NO: 10786 - RNA, 83 nt, Homo sapiens
  source 1..83: mol_type = other RNA
ctcggcgcggggcgcgggctcccctggcacggccgcccggcgcccggccgctccgccacatctgcagctcgggcagggaaggt

SEQ ID NO: 10787 - RNA, 201 nt, Homo sapiens
  source 1..201: mol_type = other RNA
ctcggcgcggggcgcgggctcccgcggccgccccgggtctgctgcgcgggcaggcagacccaccggcagacaggcggaccgggcgctcggctgtcgctgttctccgcgcggcggctgcggggcttctgacttggagaacaatgaagcgtgagctggaggggagcgagcgggccgccgggagcgcactgtgtacaaacagag

SEQ ID NO: 10788 - RNA, 214 nt, Homo sapiens
  source 1..214: mol_type = other RNA
ctcggcgcggggcgcgggctcccgcggccgccccgggtctgctgcgcgggcaggcagacccaccggcagacaggcggaccgggcgctcggctgtcgctgttctccgcgcggcggctgcggggcttctgacttggagaacaatgaagcgtgagctggaggggagcgagcgggccgccgggagcgcactgtgtacaaacagaggcggcgtgcgtgt

SEQ ID NO: 10789 - RNA, 319 nt, Homo sapiens
  source 1..319: mol_type = other RNA
ctcggcgcggggcgcgggctcctttctctgctccggaggcgctcgactctgctccccgccggcctccccggcctcccggcctccgcacctccctccggcgccgctcagcaggcagagcgcgcgggggcgcagcgcccggccatgccccgggcgggacgcgaggtctggagcccgcggtggatgaggagcctcggaaggcgaagagaagccgagccggtcagccgaggctgccagtcgcggcggattctgctcctccgccgccgccgcctcaaagcgcaccattcagcacatcctctatacacagagggagagagcgagt

SEQ ID NO: 10790 - RNA, 930 nt, Homo sapiens
  source 1..930: mol_type = other RNA
ctcgggagggcatgggccaggccttggtcactgccctcagggtggggacagacacactcagaacggacttagcacgtgcctccatcagggcgtgtcaggaagcatgttgtggagaaggtggcgtttactctggactttgaagaacaaggcgaggtagccagggacaggggctgagccttcctggcaggggttacagcctagcaaaagcccagaggggtagttaaaaataaagagtgcttcaaacgctcaataatggaaccattgtgctggccacatcctcctgagaacctcagccgctgagccaggcccttgaagtcggcagtggcttcaggtgggaagctgcatctgtgcttgcagaacctttacttgtctaagttgcctcctctctgataagagcatgtagggtatgaatgagaaagagatttcacatgtgctgagcgggcatcacctcatttcatccttacatgcgtcttctgggggctgtgatatctttagcccactctgcaggttggcatactgaggcttcttacattatctgcaaagtggcagagttgagacttgaacctgggtctggtccaaaatctgtgcttttaagctctctgtcatcccagttctcgaaaagcccagaattttctgttgaactcctggggatgagtttagtgatgtgctcgtacatattgaataaccagctctctggaagaaaaaagaggcttgattggtagcgtattccgatgtccaaggggtaaatactcccactgtggctgacatggagctatcagtgtgacattcttgaatatggagttgggaagagatgagcacagttggttcttgcaagtaggtaagggccagctccagcgtgtcactgggtaaatgtccctgcctcccccccgagcccagtatggccagtaaaggcctttagacatgtctaag

SEQ ID NO: 10791 - RNA, 1079 nt, Homo sapiens
  source 1..1079: mol_type = other RNA
ctcgtgggctctggccacggcctccagtttgtcaaacaggtctgcctccaccattgagatctcgtcaatgaccaaccgctggcagttcagccagccctgccgcacgcctggcctttgggccagggccacacactgggctagaggagcctggcctgagccgatgcctgcaaaggcatggagggtggtgcccccgatgtggcaggctgccaccccagtgctggcagtggccacagtgcctgtggggggcagtgagcccaggattcgctttagcagatatgacttccctgttcctgcactcccagtgaagaagatgctctggcctttcaggacggccctcagcacagcagcctgttcctcagaaagctgtggcttggtggagggcaagctcagcctcttcacaggcaggggccaccttggggcttctgtgctaggctcggccccagcctggggctccacaggccgcttcaccagcgtagtgtccggaacccgggtggccgccctgagccgccgctcctcgggctgcacagggctgatggtgacgaagtcgcggggccgcgggcccagcagctgcgctcgggcggaggccggcccgggacccggggccgcagccagcttgaggcgcaatgtgcgcaggaagcggcgcaggcggtctggggggcagtccgagagcagcagctgcactgcgccggccccgggggtgtcgtgggcggggagccgcagggtgctgcgcccggcctcggcgaaacgcgtgaagaggcgcgcggcgcgcagaggaaagcagcgcggccgccccgcgggccctggcgcttgcagccgcagcatcaactcgcggcgctcgttgcgacccaggctcagctccgcggtgcgcagggcctggcgccttcgcggctgcccgcccgggctcagctcctccacagccacgcggcaccgcagctccgagtcctcatattcccctgccgccgcctctatgcccgagagcatcgtcaccgcctctgctggtctctgggttcgggcagacactcacttgtgccgacactcagatgaacaagcagatcgtagccggcctgtggctaagctcc

SEQ ID NO: 10792 - RNA, 1024 nt, Homo sapiens
  source 1..1024: mol_type = other RNA
ctcgtgggctctggccacggcctccagtttgtcaaacaggtctgcctccaccattgagatctcgtcaatgaccaaccgctggcagttcagccagccctgccgcacgcctggcctttgggccagggccacacactgggctagaggagcctggcctgagccgatgcctgcaaaggcatggagggtggtgcccccgatgtggcaggctgccaccccagtgctggcagtggccacagtgcctgtggggggcagtgagcccaggattcgctttagcagatatgacttccctgttcctgcactcccagtgaagaagatgctctggcctttcaggacggccctcagcacagcagcctgttcctcagaaagctgtggcttggtggagggcaagctcagcctcttcacaggcaggggccaccttggggcttctgtgctaggctcggccccagcctggggctccacaggccgcttcaccagcgtagtgtccggaacccgggtggccgccctgagccgccgctcctcgggctgcacagggctgatggtgacgaagtcgcggggccgcgggcccagcagctgcgctcgggcggaggccggcccgggacccggggccgcagccagcttgaggcgcaatgtgcgcaggaagcggcgcaggcggtctggggggcagtccgagagcagcagctgcactgcgccggccccgggggtgtcgtgggcggggagccgcagggtgctgcgcccggcctcggcgaaacgcgtgaagaggcgcgcggcgcgcagaggaaagcagcgcggccgccccgcgggccctggcgcttgcagccgcagcatcaactcgcggcgctcgttgcgacccaggctcagctccgcggtgcgcagggcctggcgccttcgcggctgcccgcccgggctcagctcctccacagccacgcggcaccgcagctccgagtcctcatattcccctgccgccgcctctatgcccgagagcatcgtcaccgcctctgctggtctgaagttaggagttctgagacca

SEQ ID NO: 10793 - RNA, 1192 nt, Homo sapiens
  source 1..1192: mol_type = other RNA
ctcgtgggctctggccacggcctccagtttgtcaaacaggtctgcctccaccattgagatctcgtcaatgaccaaccgctggcagttcagccagccctgccgcacgcctggcctttgggccagggccacacactgggctagaggagcctggcctgagccgatgcctgcaaaggcatggagggtggtgcccccgatgtggcaggctgccaccccagtgctggcagtggccacagtgcctgtggggggcagtgagcccaggattcgctttagcagatatgacttccctgttcctgcactcccagtgaagaagatgctctggcctttcaggacggccctcagcacagcagcctgttcctcagaaagctgtggcttggtggagggcaagctcagcctcttcacaggcaggggccaccttggggcttctgtgctaggctcggccccagcctggggctccacaggccgcttcaccagcgtagtgtccggaacccgggtggccgccctgagccgccgctcctcgggctgcacagggctgatggtgacgaagtcgcggggccgcgggcccagcagctgcgctcgggcggaggccggcccgggacccggggccgcagccagcttgaggcgcaatgtgcgcaggaagcggcgcaggcggtctggggggcagtccgagagcagcagctgcactgcgccggccccgggggtgtcgtgggcggggagccgcagggtgctgcgcccggcctcggcgaaacgcgtgaagaggcgcgcggcgcgcagaggaaagcagcgcggccgccccgcgggccctggcgcttgcagccgcagcatcaactcgcggcgctcgttgcgacccaggctcagctccgcggtgcgcagggcctggcgccttcgcggctgcccgcccgggctcagctcctccacagccacgcggcaccgcagctccgagtcctcatattcccctgccgccgcctctatgcccgagagcatcgtcaccgcctctgctggtctgctcgcttaatcactccatggggcttagctactacaccacactgctcccagtctgttagcggtagagggtgatgactgaaagttgtccaggttcttggcgttttgaacaaagaattggacaaaatgcccatcaaagcaaagaaagaatgaagcaacaaaagaacaaaagcaggaattttttgaaaacgaa

SEQ ID NO: 10794 - RNA, 1055 nt, Homo sapiens
  source 1..1055: mol_type = other RNA
ctcgtgggctctggccacggcctccagtttgtcaaacaggtctgcctccaccattgagatctcgtcaatgaccaaccgctggcagttcagccagccctgccgcacgcctggcctttgggccagggccacacactgggctagaggagcctggcctgagccgatgcctgcaaaggcatggagggtggtgcccccgatgtggcaggctgccaccccagtgctggcagtggccacagtgcctgtggggggcagtgagcccaggattcgctttagcagatatgacttccctgttcctgcactcccagtgaagaagatgctctggcctttcaggacggccctcagcacagcagcctgttcctcagaaagctgtggcttggtggagggcaagctcagcctcttcacaggcaggggccaccttggggcttctgtgctaggctcggccccagcctggggctccacaggccgcttcaccagcgtagtgtccggaacccgggtggccgccctgagccgccgctcctcgggctgcacagggctgatggtgacgaagtcgcggggccgcgggcccagcagctgcgctcgggcggaggccggcccgggacccggggccgcagccagcttgaggcgcaatgtgcgcaggaagcggcgcaggcggtctggggggcagtccgagagcagcagctgcactgcgccggccccgggggtgtcgtgggcggggagccgcagggtgctgcgcccggcctcggcgaaacgcgtgaagaggcgcgcggcgcgcagaggaaagcagcgcggccgccccgcgggccctggcgcttgcagccgcagcatcaactcgcggcgctcgttgcgacccaggctcagctccgcggtgcgcagggcctggcgccttcgcggctgcccgcccgggctcagctcctccacagccacgcggcaccgcagctccgagtcctcatattcccctgccgccgcctctatgcccgagagcatcgtcaccgcctctgctggtttgtgccgacactcagatgaacaagcagatcgtagccggcctgtggctaagctcc

SEQ ID NO: 10795 - RNA, 1221 nt, Homo sapiens
  source 1..1221: mol_type = other RNA
ctcgtgggctctggccacggcctccagtttgtcaaacaggtctgcctccaccattgagatctcgtcaatgaccaaccgctggcagttcagccagccctgccgcacgcctggcctttgggccagggccacacactgggctagaggagcctggcctgagccgatgcctgcaaaggcatggagggtggtgcccccgatgtggcaggctgccaccccagtgctggcagtggccacagtgcctgtggggggcagtgagcccaggattcgctttagcagatatgacttccctgttcctgcactcccagtgaagaagatgctctggcctttcaggacggccctcagcacagcagcctgttcctcagaaagctgtggcttggtggagggcaagctcagcctcttcacaggcaggggccaccttggggcttctgtgctaggctcggccccagcctggggctccacaggccgcttcaccagcgtagtgtccggaacccgggtggccgccctgagccgccgctcctcgggctgcacagggctgatggtgacgaagtcgcggggccgcgggcccagcagctgcgctcgggcggaggccggcccgggacccggggccgcagccagcttgaggcgcaatgtgcgcaggaagcggcgcaggcggtctggggggcagtccgagagcagcagctgcactgcgccggccccgggggtgtcgtgggcggggagccgcagggtgctgcgcccggcctcggcgaaacgcgtgaagaggcgcgcggcgcgcagaggaaagcagcgcggccgccccgcgggccctggcgcttgcagccgcagcatcaactcgcggcgctcgttgcgacccaggctcagctccgcggtgcgcagggcctggcgccttcgcggctgcccgcccgggctcagctcctccacagccacgcggcaccgcagctccgagtcctcatattcccctgccgccgcctctatgcccgagagcatcgtcaccgcctctgctggtttgtgccgacactcagatgaacaagcagatcgtagccggcctgtggctaagctccgaaactagaaatttttcaaatgctagaggcagaaaatcacccaatcaccgactggatctttaaattctccagccactcagaggtaggggcgtaacaatgggcgtgtctttctttgcgtctctactccaggagcttgggctgtaccaattgcctgctagaggaagga

SEQ ID NO: 10796 - RNA, 3408 nt, Homo sapiens
  source 1..3408: mol_type = other RNA
ctctagagggaagcactttctgaaccagtaatagttgcaacttcagcagagaaagcttgctgattaagactgcttgtttcagaatctatatgaagagtagttagactagccacttcctgctcttcagcactctgatgatggccagaacctgaatccacatcagcagaggacgtaaccccagtgtcggctccaaagccaaaattgtcaaatttttggccatcatattggaaagcgctgaaagaatccgaatgactatctgagctgataagatcactgctccctgcactggcaggagaagtccattctgagggcacacctgggtcatcaatagggcgcatctggttctgcttgtttagaatatcagggaggtctttgggaatttccaggctgcctggactacttcctcttcttgtcatagtcgaggcattaccacttcgaagtcattctgctataaactcatccatcagatcaggaacattagcactgctgctgccaatatcactattaagaggaggcagtttttggctcatgtcctctttattgactttggctcgttcaacagtgaatggttccaagatgtcagaagtgctgctacttcaaggcaatggctgctcctcattcaaagcaccaaaaacttcatttccagtttcttcactttgtgaaaaatgtctgactctagttgagcggggaagtatttgagcatcatcaatatcgacagttttttgccgtactatactcctcgccttttcggttcctggagaaccagtggttgttgcactcctctgtctcattggggcttggccaggctgatcacgactccatcctctagaaaatgacttgtcaactgaaactttctgaaattcatgtccaactcctttccctttgtgctttttttgtttctgttcactcagcttatccaatggtaaatcactgagatccaaactatataaattcctagctaaaactttagttaatgtctccatagtcagtgaccactcagtggccaactcttcccaataggtcaacgatgacaatactgacagtaagtcatcccaaagttctcgggagatgtacacatttaggtttgctttgatccaggcaactataagggtctggaaaagtggtcctgcaagtcgacctgccaaggtcatattttttttcccttggaactgtagaaaagcttgtgatggcatcttcagtacagattccgtgactctgagcaacacaagcagcatgtgttcccaagtctttttgtccattgatacttgtacaaccatgtaccgataaatgttaagaatgcgtttacacatatctgtgtgttcatccagaagattttttatttcatttgcaggttcaagaagaaatatatttgatgagtttataataaacacctgcaaaactgcctgggtaccagctcgtatgttttgttctgtggcttcttcagaggtgttatgaagagcaccttggtaggagccgttttttgcccaactggaatttcgaacatgatcagcagtattggtcccattttcctcttctcttttttctccttcttccattgaaatatcatggtctgtgacattttcaatgcaagggaggtctgaagaagtgatcacaatttcttcaggctcttgcatgaacaaaggtttttcctcttgttggatccattcttgatatacttttaccacttttctcatagctgctgcttcacaaattggtaataaaaatgcctgacgaaatatctctgtcacaaagtttacattactccttttagaagaaaaaactctgcgaactatttcaatgtctgtgagatgttcttcatcaatactacagagactagatgagctaggttctcgctccgtgagagtgcttgtattggaatgagactgttcgggttctgtagttctgtctgctttatcagcattatcatttttgctttcttctctggatactaaactagcagctgctctctgaatattctttggcaagacttcaccttccatcccaggaatatgaggtcctgtatgtggttttggctccagccagaaagaaaccagccaacgaatgacaataacacgagccttaatgaaaggctcctttgtacaatagattgcttcattggtttcagcatctttctttatcatgacataatgtggctttggtctcatctgcgggatgtcaagtataggatgatataaactgttttccttacagatgtttggaaaaatataaggcaagtaatatttcttaaaatgtgaaaacaaaaatgaaaatcccctttcttggttttctttgttcttccattctaaactttttacctgaatgactatgtattttagaagtgcttcaagaaaatagcttgtgagatcttcttgccctttatctcctgattgtggggggacaagaggagtgatttcttctatagtgacttgagtttcttaaaggttgagtggaggattaatgagattatctaaagttcgaggtccatgttcagactgtggtgctgaaaatccagggattaagcatgaaaacatccagagctgttctttgctacagttattctgaagagcttgcaaccatagtaagaaaagacgaacaccttcccgcctaatctttaaggagtctcctgtgtgaagtagcttctttaaatcaatccaatattatgaaactgccatggctgatgaattctttctggaagaagttgtaaaattttctcaaaaataaaaagtatagcatccagttcctctctttgagacttgtgacctttctgtttaagactagcttcgatagtcacaaaattttcaaagaacacatagtatatatgtaaaaaatgttgtcgaaaaactgtttaagatcaatagattctgcattctttttttcactaaataaacatcactttccaaaacaaatacgcatcaggaagacagctcgagataaactctgaactaggattcaggcatctggatgaatgcatcttcttcagccagttccaccattaactcgatgacgatgcgcaggtgcttgaggcgagtcagtgcgtccttcttggtgtctagcaccttctgggtggacttcttcacgtccccgtgcggcttcttggagaacatcctgccgctgccactgccactgccactgccactgccacagccggctcccagcggcagaaagtggagggagtggacggggaggagactagccagagaggctcattagctccccagccttgcgggccagggcagagccgactcctccccgatccaggccagggccgccacctccacccgcctcgcgccgcggctccaaggcaccttcggccccagctccaatatggcggatccctctcccggccctgcacggagcgaggtagacccgggctggccgcctgccgccgccgctcgtctccagcggccg

SEQ ID NO: 10797 - RNA, 4530 nt, Homo sapiens
  source 1..4530: mol_type = other RNA
ctctagagggaagcactttctgaaccagtaatagttgcaacttcagcagagaaagcttgctgattaagactgcttgtttcagaatctatatgaagagtagttagactagccacttcctgctcttcagcactctgatgatggccagaacctgaatccacatcagcagaggacgtaaccccagtgtcggttccaaagccaaaattgtcaaattttcggccatcatattggaaagcgctgaaagaatccgaatgactatctgagctgataagatcactgctccctgcactggcaggagaagtccattctgagggcacacctgggtcatcaatagggcgcatctggttctgcttgtttagaatatcagggaggtctttgggaatttccaggctgcctggactacttcctcttcttgtcatagtcgaggcattaccacttcgaagtcgttctgctataaactcatccatcagatcaggaacattagcactgctgccgccaatatcactattaagaggaggcagtttttggctcatgtcctctttattgactgcagctttccttccaaaatagcccattacatgactgtacagatccctcagtggagcctctggtggcattctgttctgcctctgtggggaaacatttgccttcggcttcgaaagagcatgtacaacagttttataaacgccacccagggagccctgctgtagtcctgcctcatgacttgatgacctaagagtactacgactacctaattgactacttgcaattccttctttttgtaatatggtggtgggaatctctgtggattccttcactgttttgctgcttactgatgcagtaccaagtgtatctagaggtctgtacacaccaggttttactagctctgtagcactatttgtgctggtatgggtgttgctagtgctgctattgctgctaccactactaaagccaccgagcttccgcagtctcatcttccatggagcctctttgttttccagaggattataaaactgaacggactcagtggatggcctaaaagtaacatgaacactatttcgttttttagtagcaattttcatgattttggctctatgagttactgtttcagacaagctccttttagttggagaaagtttgctagtacttgtaacatgaggcattctgcggttaacaggtgcttttagtgttgctttcttggcacgcataacatgtgggacagtgattttttcattaatttgcacactcttaagcttttcaactagtgttacatcaacacaagcatctaattctgtggctgcttgtctgtacagatgtttccttttttctttatcacaagggctatctaaactaggctctgatggctgtttatcagtgtttagttgcttagatttttcagaagtttgtgttctaaaaaaactgtctgactggttaggtgcgatattactcatgaagacagctgagtttggttctttctgaaactgtaggttttcaggagtcccaacaaaagaggtgatattttctgattcagtttcctgatctgtgcattctaatttatctaaggataatctttcacccctatttactgcaatagtcacttcctgagaagctgggtctttccctgtctcatttttactatgattttcctggttttccttaaaatattctttcagggtggaaagaagatcatcatctccttcaaggtcaatgtactggatttgttcaaaagctgaatctgcaagttctactggacctattaaatgacaaagatggtcatatatgctatcaccaacttccagagaagactctctactatgagtatcagtgatgtggctttcagtggatctagttattgaagaagcctctgtggaactctgcaagcttggtgcatgacgggatgaactgtcaatgacaggaactgcacctttggctcgttcaacagtgaatggttccaagatgtcagaagtgctgctacttcgaggcaatggctgctcctcattcaaagcaccaaaaacttcatttccagtttcttcactttgtgaaaaatgtctgactctagttgagcggggaagtatttgagcatcatcaatatcgacagttttttgccgtactatactcctcgccttttcggttcctggagaaccagtggttgttgcactcctctgtctcattggggcttggccaggctgatcacgactccatcctctagaaaatgacttgtcaactgaaactttctgaaattcatgtccaactcctttccctttgtgctttttttgtttctgttcactcagcttatccaatggtaaatcactgagatccaaactatataaattcctagctaaaactttagttaatgtctccatagtcagtgaccactcagtggccaactcttcccaataggtcagcgatgacaatactgacagtaagtcatcccaaagttctcgggagatgtacacatttaggtttgctttgatccaggcaactataagggtctggaaaagtggtcctgcaagtcgacctgccaaggtcatattttttttcccttggaactgtagaaaagcttgtgatggcatcttcagtacagattccgtgactctgagcaacacaagcagcatctgttcccaagtctttttgtccattgatacttgtacaaccatgtaccgataaatgttaagaatgcgtttacacatatctgtgtgttcatccagaagattttttatttcatttgcaggttcaagaagaaatatatttgatgagtttataataaacacctgcaaaactgcctgggtaccagctcgtatgttttgttctgtggcttcttcagaggcgttatgaagagcaccttggtaggagccgttttttgcccaactggaatttcgaacatgatcagcagtattggtcccattttcctcttctcttttttctccttcttccattgaaatatcatggtctgtgacattttcaatgcaagggaggtctgaagaagtgatcacaatttcttcaggctcttgcatgaacaaaggtttttcctcttgttggatccattcttgatatacttttaccacttttctcatagctgctgcttcacaaattggtaataaaaatgcctgacgaaatatctctgtcacaaagtttacattactccttttagaagaaaaaactctgcgaactatttcaatgtctgtgagatgttcttcatcaatactacagagactagatgagctaggttctcgctccgtgagagtgcttgtattggaatgagactgttcgggttctgtagttctgtctgttttatcagcattatcatttttgctttcttctctggatactaaactagcagctgctctctgaatattctttggcaagacttcaccttccatcccaggaatatgaggtcctgtatgtggttttggctccagccagaaagaaaccagccaacgaatgacaataacacgagccttaatgaaaggctcctttgtacaatagattgcttcattggtttcagcatctttctttatcacgacataatgtggctttggtctcatctgcgggatgtcaagtataggatgatataaactgttttccttacagatgtttggaaaaatataaggcaagtaatatttcttaaaatgtgaaaacaaaaatgaaaatcccctttcttggttttctttgttcttccattctaaactttttacctgaatgactatgtattttagaagtgcttcaagaaaatagcttgtgagatcttcttgccctttatctcctgattgtggggggacaagaggagtgatttcttctatagtgacttgagtttcttgaaggttgagtggaggattaatgagattatctaaagttcgaggtccatgttcagactgtggtgctgaaaatccagggattaagcatgaaaacatccagagctgttctttgctacagttattctgaagagcttgcaaccatagtaagaaaagacgaacaccttcccgcctaatctttaaggagtttcctgtgtgaagtagcttctttaaaatcaatccaatactatgaaactgccatcgctgatgaattctttctggaagaagttgtaaaattttctcaaaaataaaaagtatagcatccaattcctctctttgagacttgtgacctttctgtttaagactagcttcaatagtcacaaaattttcaaagaacacatagtatatatgtgaaaaatgttggtcgaaaaactgtttaagatcaatagattctgcattctcgatgacgatgcgcaggtgcttgaggcgagtcagtgcgtccttcttggtgtctagcaccttctgggtggacttcttcacgtccccgtgcggcttcttggagaacatcctgtcgctgccactgccactgccactgccacagccggctcccagccgggtcccggcggcagaaagtggagggagtggacggggaggagactagccagagaggctcattagctccccagccttgcgggccagggcagagccgactccttcccgatccaggccagggccgccacct

SEQ ID NO: 10798 - RNA, 4815 nt, Homo sapiens
  source 1..4815: mol_type = other RNA
ctctagagggaagcactttctgaaccagtaatagttgcaacttcagcagagaaagcttgctgattaagactgcttgtttcagaatctatatgaagagtagttagactagccacttcctgctcttcagcactctgatgatggccagaacctgaatccacatcagcagaggacgtaaccccagtgtcggttccaaagccaaaattgtcaaattttcggccatcatattggaaagcgctgaaagaatccgaatgactatctgagctgataagatcactgctccctgcactggcaggagaagtccattctgagggcacacctgggtcatcaatagggcgcatctggttctgcttgtttagaatatcagggaggtctttgggaatttccaggctgcctggactacttcctcttcttgtcatagtcgaggcattaccacttcgaagtcgttctgctataaactcatccatcagatcaggaacattagcactgctgccgccaatatcactattaagaggaggcagtttttggctcatgtcctctttattgactgcagctttccttccaaaatagcccattacatgactgtacagatccctcagtggagcctctggtggcattctgttctgcctctgtggggaaacatttgccttcggcttcgaaagagcatgtacaacagttttataaacgccacccagggagccctgctgtagtcctgcctcatgacttgatgacctaagagtactacgactacctaattgactacttgcaattccttctttttgtaatatggtggtgggaatctctgtggattccttcactgttttgctgcttactgatgcagtaccaagtgtatctagaggtctgtacacaccaggttttactagctctgtagcactatttgtgctggtatgggtgttgctagtgctgctattgctgctaccactactaaagccaccgagcttccgcagtctcatcttccatggagcctctttgttttccagaggattataaaactgaacggactcagtggatggcctaaaagtaacatgaacactatttcgttttttagtagcaattttcatgattttggctctatgagttactgtttcagacaagctccttttagttggagaaagtttgctagtacttgtaacatgaggcattctgcggttaacaggtgcttttagtgttgctttcttggcacgcataacatgtgggacagtgattttttcattaatttgcacactcttaagcttttcaactagtgttacatcaacacaagcatctaattctgtggctgcttgtctgtacagatgtttccttttttctttatcacaagggctatctaaactaggctctgatggctgtttatcagtgtttagttgcttagatttttcagaagtttgtgttctaaaaaaactgtctgactggttaggtgcgatattactcatgaagacagctgagtttggttctttctgaaactgtaggttttcaggagtcccaacaaaagaggtgatattttctgattcagtttcctgatctgtgcattctaatttatctaaggataatctttcacccctatttactgcaatagtcacttcctgagaagctgggtctttccctgtctcatttttactatgattttcctggttttccttaaaatattctttcagggtggaaagaagatcatcatctccttcaaggtcaatgtactggatttgttcaaaagctgaatctgcaagttctactggacctattaaatgacaaagatggtcatatatgctatcaccaacttccagagaagactctctactatgagtatcagtgatgtggctttcagtggatctagttattgaagaagcctctgtggaactctgcaagcttggtgcatgacgggatgaactgtcaatgacaggaactgcacctttggctcgttcaacagtgaatggttccaagatgtcagaagtgctgctacttcgaggcaatggctgctcctcattcaaagcaccaaaaacttcatttccagtttcttcactttgtgaaaaatgtctgactctagttgagcggggaagtatttgagcatcatcaatatcgacagttttttgccgtactatactcctcgccttttcggttcctggagaaccagtggttgttgcactcctctgtctcattggggcttggccaggctgatcacgactccatcctctagaaaatgacttgtcaactgaaactttctgaaattcatgtccaactcctttccctttgtgctttttttgtttctgttcactcagcttatccaatggtaaatcactgagatccaaactatataaattcctagctaaaactttagttaatgtctccatagtcagtgaccactcagtggccaactcttcccaataggtcagcgatgacaatactgacagtaagtcatcccaaagttctcgggagatgtacacatttaggtttgctttgatccaggcaactataagggtctggaaaagtggtcctgcaagtcgacctgccaaggtcatattttttttcccttggaactgtagaaaagcttgtgatggcatcttcagtacagattccgtgactctgagcaacacaagcagcatctgttcccaagtctttttgtccattgatacttgtacaaccatgtaccgataaatgttaagaatgcgtttacacatatctgtgtgttcatccagaagattttttatttcatttgcaggttcaagaagaaatatatttgatgagtttataataaacacctgcaaaactgcctgggtaccagctcgtatgttttgttctgtggcttcttcagaggcgttatgaagagcaccttggtaggagccgttttttgcccaactggaatttcgaacatgatcagcagtattggtcccattttcctcttctcttttttctccttcttccattgaaatatcatggtctgtgacattttcaatgcaagggaggtctgaagaagtgatcacaatttcttcaggctcttgcatgaacaaaggtttttcctcttgttggatccattcttgatatacttttaccacttttctcatagctgctgcttcacaaattggtaataaaaatgcctgacgaaatatctctgtcacaaagtttacattactccttttagaagaaaaaactctgcgaactatttcaatgtctgtgagatgttcttcatcaatactacagagactagatgagctaggttctcgctccgtgagagtgcttgtattggaatgagactgttcgggttctgtagttctgtctgttttatcagcattatcatttttgctttcttctctggatactaaactagcagctgctctctgaatattctttggcaagacttcaccttccatcccaggaatatgaggtcctgtatgtggttttggctccagccagaaagaaaccagccaacgaatgacaataacacgagccttaatgaaaggctcctttgtacaatagattgcttcattggtttcagcatctttctttatcacgacataatgtggctttggtctcatctgcgggatgtcaagtataggatgatataaactgttttccttacagatgtttggaaaaatataaggcaagtaatatttcttaaaatgtgaaaacaaaaatgaaaatcccctttcttggttttctttgttcttccattctaaactttttacctgaatgactatgtattttagaagtgcttcaagaaaatagcttgtgagatcttcttgccctttatctcctgattgtggggggacaagaggagtgatttcttctatagtgacttgagtttcttgaaggttgagtggaggattaatgagattatctaaagttcgaggtccatgttcagactgtggtgctgaaaatccagggattaagcatgaaaacatccagagctgttctttgctacagttattctgaagagcttgcaaccatagtaagaaaagacgaacaccttcccgcctaatctttaaggagtttcctgtgtgaagtagcttctttaaaatcaatccaatactatgaaactgccatcgctgatgaattctttctggaagaagttgtaaaattttctcaaaaataaaaagtatagcatccaattcctctctttgagacttgtgacctttctgtttaagactagcttcaatagtcacaaaattttcaaagaacacatagtatatatgtgaaaaatgttggtcgaaaaactgtttaagatcaatagattctgcattctcgatgacgatgcgcaggtgcttgaggcgagtcagtgcgtccttcttggtgtctagcaccttctgggtggacttcttcacgtccccgtgcggcttcttggagaacatcctgtcgctgccactgccactgccactgccacagccggctcccagccgggtcccggcggcagaaagtggagggagtggacggggaggagactagccagagaggctcattagctccccagccttgcgggccagggcagagccgactccttcccgatccaggccagggccgccacctccacccgcctcgcgccgcggctccaaggcaccttcggccccagctccaatatggcggatccctctcccggccctgcacggagcgaggcagacccgggctggccgcctgccgccgccgctcgtctccagcggccgccgctcgccgccacaggccggggccccggacccagagccacgaaggtggagctctcggcggcaggagcacaactctctccctgaggcccccttaaggttgaagcttctttagcagcttacaccctgcagaggccgaaacggagacgagtgt

SEQ ID NO: 10799 - RNA, 4671 nt, Homo sapiens
  source 1..4671: mol_type = other RNA
ctctagagggaagcactttctgaaccagtaatagttgcaacttcagcagagaaagcttgctgattaagactgcttgtttcagaatctatatgaagagtagttagactagccacttcctgctcttcagcactctgatgatggccagaacctgaatccacatcagcagaggacgtaaccccagtgtcggttccaaagccaaaattgtcaaattttcggccatcatattggaaagcgctgaaagaatccgaatgactatctgagctgataagatcactgctccctgcactggcaggagaagtccattctgagggcacacctgggtcatcaatagggcgcatctggttctgcttgtttagaatatcagggaggtctttgggaatttccaggctgcctggactacttcctcttcttgtcatagtcgaggcattaccacttcgaagtcgttctgctataaactcatccatcagatcaggaacattagcactgctgccgccaatatcactattaagaggaggcagtttttggctcatgtcctctttattgactgcagctttccttccaaaatagcccattacatgactgtacagatccctcagtggagcctctggtggcattctgttctgcctctgtggggaaacatttgccttcggcttcgaaagagcatgtacaacagttttataaacgccacccagggagccctgctgtagtcctgcctcatgacttgatgacctaagagtactacgactacctaattgactacttgcaattccttctttttgtaatatggtggtgggaatctctgtggattccttcactgttttgctgcttactgatgcagtaccaagtgtatctagaggtctgtacacaccaggttttactagctctgtagcactatttgtgctggtatgggtgttgctagtgctgctattgctgctaccactactaaagccaccgagcttccgcagtctcatcttccatggagcctctttgttttccagaggattataaaactgaacggactcagtggatggcctaaaagtaacatgaacactatttcgttttttagtagcaattttcatgattttggctctatgagttactgtttcagacaagctccttttagttggagaaagtttgctagtacttgtaacatgaggcattctgcggttaacaggtgcttttagtgttgctttcttggcacgcataacatgtgggacagtgattttttcattaatttgcacactcttaagcttttcaactagtgttacatcaacacaagcatctaattctgtggctgcttgtctgtacagatgtttccttttttctttatcacaagggctatctaaactaggctctgatggctgtttatcagtgtttagttgcttagatttttcagaagtttgtgttctaaaaaaactgtctgactggttaggtgcgatattactcatgaagacagctgagtttggttctttctgaaactgtaggttttcaggagtcccaacaaaagaggtgatattttctgattcagtttcctgatctgtgcattctaatttatctaaggataatctttcacccctatttactgcaatagtcacttcctgagaagctgggtctttccctgtctcatttttactatgattttcctggttttccttaaaatattctttcagggtggaaagaagatcatcatctccttcaaggtcaatgtactggatttgttcaaaagctgaatctgcaagttctactggacctattaaatgacaaagatggtcatatatgctatcaccaacttccagagaagactctctactatgagtatcagtgatgtggctttcagtggatctagttattgaagaagcctctgtggaactctgcaagcttggtgcatgacgggatgaactgtcaatgacaggaactgcacctttggctcgttcaacagtgaatggttccaagatgtcagaagtgctgctacttcgaggcaatggctgctcctcattcaaagcaccaaaaacttcatttccagtttcttcactttgtgaaaaatgtctgactctagttgagcggggaagtatttgagcatcatcaatatctgaaagctcatcagaaaggggagtgagaacaatatcaggcaagaagggtttggaagtatggatcagaacaggagcacttttagcactgcgtatataggccgatggcagagcacattcaccaatggatcggcttctcatggcgacagttttttgccgtactatactcctcgccttttcggttcctggagaaccagtggttgttgcactcctctgtctcattggggcttggccaggctgatcacgactccatcctctagaaaatgacttgtcaactgaaactttctgaaattcatgtccaactcctttccctttgtgctttttttgtttctgttcactcagcttatccaatggtaaatcactgagatccaaactatataaattcctagctaaaactttagttaatgtctccatagtcagtgaccactcagtggccaactcttcccaataggtcagcgatgacaatactgacagtaagtcatcccaaagttctcgggagatgtacacatttaggtttgctttgatccaggcaactataagggtctggaaaagtggtcctgcaagtcgacctgccaaggtcatattttttttcccttggaactgtagaaaagcttgtgatggcatcttcagtacagattccgtgactctgagcaacacaagcagcatctgttcccaagtctttttgtccattgatacttgtacaaccatgtaccgataaatgttaagaatgcgtttacacatatctgtgtgttcatccagaagattttttatttcatttgcaggttcaagaagaaatatatttgatgagtttataataaacacctgcaaaactgcctgggtaccagctcgtatgttttgttctgtggcttcttcagaggcgttatgaagagcaccttggtaggagccgttttttgcccaactggaatttcgaacatgatcagcagtattggtcccattttcctcttctcttttttctccttcttccattgaaatatcatggtctgtgacattttcaatgcaagggaggtctgaagaagtgatcacaatttcttcaggctcttgcatgaacaaaggtttttcctcttgttggatccattcttgatatacttttaccacttttctcatagctgctgcttcacaaattggtaataaaaatgcctgacgaaatatctctgtcacaaagtttacattactccttttagaagaaaaaactctgcgaactatttcaatgtctgtgagatgttcttcatcaatactacagagactagatgagctaggttctcgctccgtgagagtgcttgtattggaatgagactgttcgggttctgtagttctgtctgttttatcagcattatcatttttgctttcttctctggatactaaactagcagctgctctctgaatattctttggcaagacttcaccttccatcccaggaatatgaggtcctgtatgtggttttggctccagccagaaagaaaccagccaacgaatgacaataacacgagccttaatgaaaggctcctttgtacaatagattgcttcattggtttcagcatctttctttatcacgacataatgtggctttggtctcatctgcgggatgtcaagtataggatgatataaactgttttccttacagatgtttggaaaaatataaggcaagtaatatttcttaaaatgtgaaaacaaaaatgaaaatcccctttcttggttttctttgttcttccattctaaactttttacctgaatgactatgtattttagaagtgcttcaagaaaatagcttgtgagatcttcttgccctttatctcctgattgtggggggacaagaggagtgatttcttctatagtgacttgagtttcttgaaggttgagtggaggattaatgagattatctaaagttcgaggtccatgttcagactgtggtgctgaaaatccagggattaagcatgaaaacatccagagctgttctttgctacagttattctgaagagcttgcaaccatagtaagaaaagacgaacaccttcccgcctaatctttaaggagtttcctgtgtgaagtagcttctttaaaatcaatccaatactatgaaactgccatcgctgatgaattctttctggaagaagttgtaaaattttctcaaaaataaaaagtatagcatccaattcctctctttgagacttgtgacctttctgtttaagactagcttcaatagtcacaaaattttcaaagaacacatagtatatatgtgaaaaatgttggtcgaaaaactgtttaagatcaatagattctgcattctcgatgacgatgcgcaggtgcttgaggcgagtcagtgcgtccttcttggtgtctagcaccttctgggtggacttcttcacgtccccgtgcggcttcttggagaacatcctgtcgctgccactgccactgccactgccacagccggctcccagccgggtcccggcggcagaaagtggagggagtggacggggaggagactagccagagaggctcattagctccccagccttgcgggccagggcagagccgactccttcccgatccaggccagggccgccacct

SEQ ID NO: 10800 - RNA, 4956 nt, Homo sapiens
  source 1..4956: mol_type = other RNA
ctctagagggaagcactttctgaaccagtaatagttgcaacttcagcagagaaagcttgctgattaagactgcttgtttcagaatctatatgaagagtagttagactagccacttcctgctcttcagcactctgatgatggccagaacctgaatccacatcagcagaggacgtaaccccagtgtcggttccaaagccaaaattgtcaaattttcggccatcatattggaaagcgctgaaagaatccgaatgactatctgagctgataagatcactgctccctgcactggcaggagaagtccattctgagggcacacctgggtcatcaatagggcgcatctggttctgcttgtttagaatatcagggaggtctttgggaatttccaggctgcctggactacttcctcttcttgtcatagtcgaggcattaccacttcgaagtcgttctgctataaactcatccatcagatcaggaacattagcactgctgccgccaatatcactattaagaggaggcagtttttggctcatgtcctctttattgactgcagctttccttccaaaatagcccattacatgactgtacagatccctcagtggagcctctggtggcattctgttctgcctctgtggggaaacatttgccttcggcttcgaaagagcatgtacaacagttttataaacgccacccagggagccctgctgtagtcctgcctcatgacttgatgacctaagagtactacgactacctaattgactacttgcaattccttctttttgtaatatggtggtgggaatctctgtggattccttcactgttttgctgcttactgatgcagtaccaagtgtatctagaggtctgtacacaccaggttttactagctctgtagcactatttgtgctggtatgggtgttgctagtgctgctattgctgctaccactactaaagccaccgagcttccgcagtctcatcttccatggagcctctttgttttccagaggattataaaactgaacggactcagtggatggcctaaaagtaacatgaacactatttcgttttttagtagcaattttcatgattttggctctatgagttactgtttcagacaagctccttttagttggagaaagtttgctagtacttgtaacatgaggcattctgcggttaacaggtgcttttagtgttgctttcttggcacgcataacatgtgggacagtgattttttcattaatttgcacactcttaagcttttcaactagtgttacatcaacacaagcatctaattctgtggctgcttgtctgtacagatgtttccttttttctttatcacaagggctatctaaactaggctctgatggctgtttatcagtgtttagttgcttagatttttcagaagtttgtgttctaaaaaaactgtctgactggttaggtgcgatattactcatgaagacagctgagtttggttctttctgaaactgtaggttttcaggagtcccaacaaaagaggtgatattttctgattcagtttcctgatctgtgcattctaatttatctaaggataatctttcacccctatttactgcaatagtcacttcctgagaagctgggtctttccctgtctcatttttactatgattttcctggttttccttaaaatattctttcagggtggaaagaagatcatcatctccttcaaggtcaatgtactggatttgttcaaaagctgaatctgcaagttctactggacctattaaatgacaaagatggtcatatatgctatcaccaacttccagagaagactctctactatgagtatcagtgatgtggctttcagtggatctagttattgaagaagcctctgtggaactctgcaagcttggtgcatgacgggatgaactgtcaatgacaggaactgcacctttggctcgttcaacagtgaatggttccaagatgtcagaagtgctgctacttcgaggcaatggctgctcctcattcaaagcaccaaaaacttcatttccagtttcttcactttgtgaaaaatgtctgactctagttgagcggggaagtatttgagcatcatcaatatctgaaagctcatcagaaaggggagtgagaacaatatcaggcaagaagggtttggaagtatggatcagaacaggagcacttttagcactgcgtatataggccgatggcagagcacattcaccaatggatcggcttctcatggcgacagttttttgccgtactatactcctcgccttttcggttcctggagaaccagtggttgttgcactcctctgtctcattggggcttggccaggctgatcacgactccatcctctagaaaatgacttgtcaactgaaactttctgaaattcatgtccaactcctttccctttgtgctttttttgtttctgttcactcagcttatccaatggtaaatcactgagatccaaactatataaattcctagctaaaactttagttaatgtctccatagtcagtgaccactcagtggccaactcttcccaataggtcagcgatgacaatactgacagtaagtcatcccaaagttctcgggagatgtacacatttaggtttgctttgatccaggcaactataagggtctggaaaagtggtcctgcaagtcgacctgccaaggtcatattttttttcccttggaactgtagaaaagcttgtgatggcatcttcagtacagattccgtgactctgagcaacacaagcagcatctgttcccaagtctttttgtccattgatacttgtacaaccatgtaccgataaatgttaagaatgcgtttacacatatctgtgtgttcatccagaagattttttatttcatttgcaggttcaagaagaaatatatttgatgagtttataataaacacctgcaaaactgcctgggtaccagctcgtatgttttgttctgtggcttcttcagaggcgttatgaagagcaccttggtaggagccgttttttgcccaactggaatttcgaacatgatcagcagtattggtcccattttcctcttctcttttttctccttcttccattgaaatatcatggtctgtgacattttcaatgcaagggaggtctgaagaagtgatcacaatttcttcaggctcttgcatgaacaaaggtttttcctcttgttggatccattcttgatatacttttaccacttttctcatagctgctgcttcacaaattggtaataaaaatgcctgacgaaatatctctgtcacaaagtttacattactccttttagaagaaaaaactctgcgaactatttcaatgtctgtgagatgttcttcatcaatactacagagactagatgagctaggttctcgctccgtgagagtgcttgtattggaatgagactgttcgggttctgtagttctgtctgttttatcagcattatcatttttgctttcttctctggatactaaactagcagctgctctctgaatattctttggcaagacttcaccttccatcccaggaatatgaggtcctgtatgtggttttggctccagccagaaagaaaccagccaacgaatgacaataacacgagccttaatgaaaggctcctttgtacaatagattgcttcattggtttcagcatctttctttatcacgacataatgtggctttggtctcatctgcgggatgtcaagtataggatgatataaactgttttccttacagatgtttggaaaaatataaggcaagtaatatttcttaaaatgtgaaaacaaaaatgaaaatcccctttcttggttttctttgttcttccattctaaactttttacctgaatgactatgtattttagaagtgcttcaagaaaatagcttgtgagatcttcttgccctttatctcctgattgtggggggacaagaggagtgatttcttctatagtgacttgagtttcttgaaggttgagtggaggattaatgagattatctaaagttcgaggtccatgttcagactgtggtgctgaaaatccagggattaagcatgaaaacatccagagctgttctttgctacagttattctgaagagcttgcaaccatagtaagaaaagacgaacaccttcccgcctaatctttaaggagtttcctgtgtgaagtagcttctttaaaatcaatccaatactatgaaactgccatcgctgatgaattctttctggaagaagttgtaaaattttctcaaaaataaaaagtatagcatccaattcctctctttgagacttgtgacctttctgtttaagactagcttcaatagtcacaaaattttcaaagaacacatagtatatatgtgaaaaatgttggtcgaaaaactgtttaagatcaatagattctgcattctcgatgacgatgcgcaggtgcttgaggcgagtcagtgcgtccttcttggtgtctagcaccttctgggtggacttcttcacgtccccgtgcggcttcttggagaacatcctgtcgctgccactgccactgccactgccacagccggctcccagccgggtcccggcggcagaaagtggagggagtggacggggaggagactagccagagaggctcattagctccccagccttgcgggccagggcagagccgactccttcccgatccaggccagggccgccacctccacccgcctcgcgccgcggctccaaggcaccttcggccccagctccaatatggcggatccctctcccggccctgcacggagcgaggcagacccgggctggccgcctgccgccgccgctcgtctccagcggccgccgctcgccgccacaggccggggccccggacccagagccacgaaggtggagctctcggcggcaggagcacaactctctccctgaggcccccttaaggttgaagcttctttagcagcttacaccctgcagaggccgaaacggagacgagtgt

SEQ ID NO: 10801 - RNA, 2634 nt, Homo sapiens
  source 1..2634: mol_type = other RNA
ctctagagggaagcactttctgaaccagtaatagttgcaacttcagcagagaaagcttgctgattaagactgcttgtttcagaatctatatgaagagtagttagactagccacttcctgctcttcagcactctgatgatggccagaacctgaatccacatcagcagaggacgtaaccccagtgtcggttccaaagccaaaattgtcaaattttcggccatcatattggaaagcgctgaaagaatccgaatgactatctgagctgataagatcactgctccctgcactggcaggagaagtccattctgagggcacacctgggtcatcaatagggcgcatctggttctgcttgtttagaatatcagggaggtctttgggaatttccaggctgcctggactacttcctcttcttgtcatagtcgaggcattaccacttcgaagtcgttctgctataaactcatccatcagatcaggaacattagcactgctgccgccaatatcactattaagaggaggcagtttttggctcatgtcctctttattgactgcagctttccttccaaaatagcccattacatgactgtacagatccctcagtggagcctctggtggcattctgttctgcctctgtggggaaacatttgccttcggcttcgaaagagcatgtacaacagttttataaacgccacccagggagccctgctgtagtcctgcctcatgacttgatgacctaagagtactacgactacctaattgactacttgcaattccttctttttgtaatatggtggtgggaatctctgtggattccttcactgttttgctgcttactgatgcagtaccaagtgtatctagaggtctgtacacaccaggttttactagctctgtagcactatttgtgctggtatgggtgttgctagtgctgctattgctgctaccactactaaagccaccgagcttccgcagtctcatcttccatggagcctctttgttttccagaggattataaaactgaacggactcagtggatggcctaaaagtaacatgaacactatttcgttttttagtagcaattttcatgattttggctctatgagttactgtttcagacaagctccttttagttggagaaagtttgctagtacttgtaacatgaggcattctgcggttaacaggtgcttttagtgttgctttcttggcacgcataacatgtgggacagtgattttttcattaatttgcacactcttaagcttttcaactagtgttacatcaacacaagcatctaattctgtggctgcttgtctgtacagatgtttccttttttctttatcacaagggctatctaaactaggctctgatggctgtttatcagtgtttagttgcttagatttttcagaagtttgtgttctaaaaaaactgtctgactggttaggtgcgatattactcatgaagacagctgagtttggttctttctgaaactgtaggttttcaggagtcccaacaaaagaggtgatattttctgattcagtttcctgatctgtgcattctaatttatctaaggataatctttcacccctatttactgcaatagtcacttcctgagaagctgggtctttccctgtctcatttttactatgattttcctggttttccttaaaatattctttcagggtggaaagaagatcatcatctccttcaaggtcaatgtactggatttgttcaaaagctgaatctgcaagttctactggacctattaaatgacaaagatggtcatatatgctatcaccaacttccagagaagactctctactatgagtatcagtgatgtggctttcagtggatctagttattgaagaagcctctgtggaactctgcaagcttggtgcatgacgggatgaactgtcaatgacaggaactgcacctttggctcgttcaacagtgaatggttccaagatgtcagaagtgctgctacttcgaggcaatggctgctcctcattcaaagcaccaaaaacttcatttccagtttcttcactttgtgaaaaatgtctgactctagttgagcggggaagtatttgagcatcatcaatatctgaaagctcatcagaaaggggagtgagaacaatatcaggcaagaagggtttggaagtatggatcagaacaggagcacttttagcactgcgtatataggccgatggcagagcacattcaccaatggatcggcttctcatggctgaaattaacttgtatccttctcaagataaccaatttaacatggaagtcttcaattcagtcatccaaccttgaagcttgctcaagtctcagtctgaatcccagaagtgattatcagcaatttgcttcaagatcatcccacttttccagtgtgcttactgctcatcactccattttccactcatagttttattttggtcaaggaaatgagtaagaagagtcttagaggtttctctatttgcaaaccagtggtacgacgaaatgctagcaagaatatctaatagctccagaatatcaagttcactatgttgctggcaatacgagtcatgtaatgactttttaaaaagcccctttcttcccaattttttattaagaaaattttcaaatgtagaaaaaattaaaaga

SEQ ID NO: 10802 - RNA, 2493 nt, Homo sapiens
  source 1..2493: mol_type = other RNA
ctctagagggaagcactttctgaaccagtaatagttgcaacttcagcagagaaagcttgctgattaagactgcttgtttcagaatctatatgaagagtagttagactagccacttcctgctcttcagcactctgatgatggccagaacctgaatccacatcagcagaggacgtaaccccagtgtcggttccaaagccaaaattgtcaaattttcggccatcatattggaaagcgctgaaagaatccgaatgactatctgagctgataagatcactgctccctgcactggcaggagaagtccattctgagggcacacctgggtcatcaatagggcgcatctggttctgcttgtttagaatatcagggaggtctttgggaatttccaggctgcctggactacttcctcttcttgtcatagtcgaggcattaccacttcgaagtcgttctgctataaactcatccatcagatcaggaacattagcactgctgccgccaatatcactattaagaggaggcagtttttggctcatgtcctctttattgactgcagctttccttccaaaatagcccattacatgactgtacagatccctcagtggagcctctggtggcattctgttctgcctctgtggggaaacatttgccttcggcttcgaaagagcatgtacaacagttttataaacgccacccagggagccctgctgtagtcctgcctcatgacttgatgacctaagagtactacgactacctaattgactacttgcaattccttctttttgtaatatggtggtgggaatctctgtggattccttcactgttttgctgcttactgatgcagtaccaagtgtatctagaggtctgtacacaccaggttttactagctctgtagcactatttgtgctggtatgggtgttgctagtgctgctattgctgctaccactactaaagccaccgagcttccgcagtctcatcttccatggagcctctttgttttccagaggattataaaactgaacggactcagtggatggcctaaaagtaacatgaacactatttcgttttttagtagcaattttcatgattttggctctatgagttactgtttcagacaagctccttttagttggagaaagtttgctagtacttgtaacatgaggcattctgcggttaacaggtgcttttagtgttgctttcttggcacgcataacatgtgggacagtgattttttcattaatttgcacactcttaagcttttcaactagtgttacatcaacacaagcatctaattctgtggctgcttgtctgtacagatgtttccttttttctttatcacaagggctatctaaactaggctctgatggctgtttatcagtgtttagttgcttagatttttcagaagtttgtgttctaaaaaaactgtctgactggttaggtgcgatattactcatgaagacagctgagtttggttctttctgaaactgtaggttttcaggagtcccaacaaaagaggtgatattttctgattcagtttcctgatctgtgcattctaatttatctaaggataatctttcacccctatttactgcaatagtcacttcctgagaagctgggtctttccctgtctcatttttactatgattttcctggttttccttaaaatattctttcagggtggaaagaagatcatcatctccttcaaggtcaatgtactggatttgttcaaaagctgaatctgcaagttctactggacctattaaatgacaaagatggtcatatatgctatcaccaacttccagagaagactctctactatgagtatcagtgatgtggctttcagtggatctagttattgaagaagcctctgtggaactctgcaagcttggtgcatgacgggatgaactgtcaatgacaggaactgcacctttggctcgttcaacagtgaatggttccaagatgtcagaagtgctgctacttcgaggcaatggctgctcctcattcaaagcaccaaaaacttcatttccagtttcttcactttgtgaaaaatgtctgactctagttgagcggggaagtatttgagcatcatcaatatctgaaattaacttgtatccttctcaagataaccaatttaacatggaagtcttcaattcagtcatccaaccttgaagcttgctcaagtctcagtctgaatcccagaagtgattatcagcaatttgcttcaagatcatcccacttttccagtgtgcttactgctcatcactccattttccactcatagttttattttggtcaaggaaatgagtaagaagagtcttagaggtttctctatttgcaaaccagtggtacgacgaaatgctagcaagaatatctaatagctccagaatatcaagttcactatgttgctggcaatacgagtcatgtaatgactttttaaaaagcccctttcttcccaattttttattaagaaaattttcaaatgtagaaaaaattaaaaga

SEQ ID NO: 10803 - RNA, 1198 nt, Homo sapiens
  source 1..1198: mol_type = other RNA
ctctagagggaagcactttctgaaccagtaatagttgcaacttcagcagagaaagcttgctgattaagactgcttgtttcagaatctatatgaagagtagttagactagccacttcctgctcttcagcactctgatgatggccagaacctgaatccacatcagcagaggacgtaaccccagtgtcggttccaaagccaaaattgtcaaattttcggccatcatattggaaagcgctgaaagaatccgaatgactatctgagctgataagatcactgctccctgcactggcaggagaagtccattctgagggcacacctgggtcatcaatagggcgcatctggttctgcttgtttagaatatcagggaggtctttgggaatttccaggctgcctggactacttcctcttcttgtcatagtcgaggcattaccacttcgaagtcgttctgctataaactcatccatcagatcaggaacattagcactgctgccgccaatatcactattaagaggaggcagtttttggctcatgtcctctttattgactgcagctttccttccaaaatagcccattacatgactgtacagatccctcagtggagcctctggtggcattctgttctgcctctttggctcgttcaacagtgaatggttccaagatgtcagaagtgctgctacttcgaggcaatggctgctcctcattcaaagcaccaaaaacttcatttccagtttcttcactttgtgaaaaatgtctgactctagttgagcggggaagtatttgagcatcatcaatatctgaaattaacttgtatccttctcaagataaccaatttaacatggaagtcttcaattcagtcatccaaccttgaagcttgctcaagtctcagtctgaatcccagaagtgattatcagcaatttgcttcaagatcatcccacttttccagtgtgcttactgctcatcactccattttccactcatagttttattttggtcaaggaaatgagtaagaagagtcttagaggtttctctatttgcaaaccagtggtacgacgaaatgctagcaagaatatctaatagctccagaatatcaagttcactatgttgctggcaatacgagtcatgtaatgactttttaaaaagcccctttcttcccaattttttattaagaaaattttcaaatgtagaaaaaattaaaaga

SEQ ID NO: 10804 - RNA, 3438 nt, Homo sapiens
  source 1..3438: mol_type = other RNA
ctctagagggaagcactttctgaaccagtaatagttgcaacttcagcagagaaagcttgctgattaagactgcttgtttcagaatctatatgaagagtagttagactagccacttcctgctcttcagcactctgatgatggccagaacctgaatccacatcagcagaggacgtaaccccagtgtcggttccaaagccaaaattgtcaaattttcggccatcatattggaaagcgctgaaagaatccgaatgactatctgagctgataagatcactgctccctgcactggcaggagaagtccattctgagggcacacctgggtcatcaatagggcgcatctggttctgcttgtttagaatatcagggaggtctttgggaatttccaggctgcctggactacttcctcttcttgtcatagtcgaggcattaccacttcgaagtcgttctgctataaactcatccatcagatcaggaacattagcactgctgccgccaatatcactattaagaggaggcagtttttggctcatgtcctctttattgactttggctcgttcaacagtgaatggttccaagatgtcagaagtgctgctacttcgaggcaatggctgctcctcattcaaagcaccaaaaacttcatttccagtttcttcactttgtgaaaaatgtctgactctagttgagcggggaagtatttgagcatcatcaatatcgacagttttttgccgtactatactcctcgccttttcggttcctggagaaccagtggttgttgcactcctctgtctcattggggcttggccaggctgatcacgactccatcctctagaaaatgacttgtcaactgaaactttctgaaattcatgtccaactcctttccctttgtgctttttttgtttctgttcactcagcttatccaatggtaaatcactgagatccaaactatataaattcctagctaaaactttagttaatgtctccatagtcagtgaccactcagtggccaactcttcccaataggtcagcgatgacaatactgacagtaagtcatcccaaagttctcgggagatgtacacatttaggtttgctttgatccaggcaactataagggtctggaaaagtggtcctgcaagtcgacctgccaaggtcatattttttttcccttggaactgtagaaaagcttgtgatggcatcttcagtacagattccgtgactctgagcaacacaagcagcatctgttcccaagtctttttgtccattgatacttgtacaaccatgtaccgataaatgttaagaatgcgtttacacatatctgtgtgttcatccagaagattttttatttcatttgcaggttcaagaagaaatatatttgatgagtttataataaacacctgcaaaactgcctgggtaccagctcgtatgttttgttctgtggcttcttcagaggcgttatgaagagcaccttggtaggagccgttttttgcccaactggaatttcgaacatgatcagcagtattggtcccattttcctcttctcttttttctccttcttccattgaaatatcatggtctgtgacattttcaatgcaagggaggtctgaagaagtgatcacaatttcttcaggctcttgcatgaacaaaggtttttcctcttgttggatccattcttgatatacttttaccacttttctcatagctgctgcttcacaaattggtaataaaaatgcctgacgaaatatctctgtcacaaagtttacattactccttttagaagaaaaaactctgcgaactatttcaatgtctgtgagatgttcttcatcaatactacagagactagatgagctaggttctcgctccgtgagagtgcttgtattggaatgagactgttcgggttctgtagttctgtctgttttatcagcattatcatttttgctttcttctctggatactaaactagcagctgctctctgaatattctttggcaagacttcaccttccatcccaggaatatgaggtcctgtatgtggttttggctccagccagaaagaaaccagccaacgaatgacaataacacgagccttaatgaaaggctcctttgtacaatagattgcttcattggtttcagcatctttctttatcacgacataatgtggctttggtctcatctgcgggatgtcaagtataggatgatataaactgttttccttacagatgtttggaaaaatataaggcaagtaatatttcttaaaatgtgaaaacaaaaatgaaaatcccctttcttggttttctttgttcttccattctaaactttttacctgaatgactatgtattttagaagtgcttcaagaaaatagcttgtgagatcttcttgccctttatctcctgattgtggggggacaagaggagtgatttcttctatagtgacttgagtttcttgaaggttgagtggaggattaatgagattatctaaagttcgaggtccatgttcagactgtggtgctgaaaatccagggattaagcatgaaaacatccagagctgttctttgctacagttattctgaagagcttgcaaccatagtaagaaaagacgaacaccttcccgcctaatctttaaggagtttcctgtgtgaagtagcttctttaaaatcaatccaatactatgaaactgccatcgctgatgaattctttctggaagaagttgtaaaattttctcaaaaataaaaagtatagcatccaattcctctctttgagacttgtgacctttctgtttaagactagcttcaatagtcacaaaattttcaaagaacacatagtatatatgtgaaaaatgttggtcgaaaaactgtttaagatcaatagattctgcattctcgatgacgatgcgcaggtgcttgaggcgagtcagtgcgtccttcttggtgtctagcaccttctgggtggacttcttcacgtccccgtgcggcttcttggagaacatcctgtcgctgccactgccactgccactgccacagccggctcccagccgggtcccggcggcagaaagtggagggagtggacggggaggagactagccagagaggctcattagctccccagccttgcgggccagggcagagccgactccttcccgatccaggccagggccgccacctccacccgcctcgcgccgcggctccaaggcaccttcggccccagctccaatatggcggatccctctcccggccctgcacggagcgaggcagacccgggctggccgcctgccgccgccgctcgtctccagcggccgccgctcgccgccacaggccggggccccggacccagagccacgaaggtggagctctcggcggcaggagcacaactctctccctgaggcccccttaaggttgaagcttctttagcagcttacaccctgcagaggccgaaacggagacgagtgt

SEQ ID NO: 10805 - RNA, 3294 nt, Homo sapiens
  source 1..3294: mol_type = other RNA
ctctagagggaagcactttctgaaccagtaatagttgcaacttcagcagagaaagcttgctgattaagactgcttgtttcagaatctatatgaagagtagttagactagccacttcctgctcttcagcactctgatgatggccagaacctgaatccacatcagcagaggacgtaaccccagtgtcggttccaaagccaaaattgtcaaattttcggccatcatattggaaagcgctgaaagaatccgaatgactatctgagctgataagatcactgctccctgcactggcaggagaagtccattctgagggcacacctgggtcatcaatagggcgcatctggttctgcttgtttagaatatcagggaggtctttgggaatttccaggctgcctggactacttcctcttcttgtcatagtcgaggcattaccacttcgaagtcgttctgctataaactcatccatcagatcaggaacattagcactgctgccgccaatatcactattaagaggaggcagtttttggctcatgtcctctttattgactttggctcgttcaacagtgaatggttccaagatgtcagaagtgctgctacttcgaggcaatggctgctcctcattcaaagcaccaaaaacttcatttccagtttcttcactttgtgaaaaatgtctgactctagttgagcggggaagtatttgagcatcatcaatatctgaaagctcatcagaaaggggagtgagaacaatatcaggcaagaagggtttggaagtatggatcagaacaggagcacttttagcactgcgtatataggccgatggcagagcacattcaccaatggatcggcttctcatggcgacagttttttgccgtactatactcctcgccttttcggttcctggagaaccagtggttgttgcactcctctgtctcattggggcttggccaggctgatcacgactccatcctctagaaaatgacttgtcaactgaaactttctgaaattcatgtccaactcctttccctttgtgctttttttgtttctgttcactcagcttatccaatggtaaatcactgagatccaaactatataaattcctagctaaaactttagttaatgtctccatagtcagtgaccactcagtggccaactcttcccaataggtcagcgatgacaatactgacagtaagtcatcccaaagttctcgggagatgtacacatttaggtttgctttgatccaggcaactataagggtctggaaaagtggtcctgcaagtcgacctgccaaggtcatattttttttcccttggaactgtagaaaagcttgtgatggcatcttcagtacagattccgtgactctgagcaacacaagcagcatctgttcccaagtctttttgtccattgatacttgtacaaccatgtaccgataaatgttaagaatgcgtttacacatatctgtgtgttcatccagaagattttttatttcatttgcaggttcaagaagaaatatatttgatgagtttataataaacacctgcaaaactgcctgggtaccagctcgtatgttttgttctgtggcttcttcagaggcgttatgaagagcaccttggtaggagccgttttttgcccaactggaatttcgaacatgatcagcagtattggtcccattttcctcttctcttttttctccttcttccattgaaatatcatggtctgtgacattttcaatgcaagggaggtctgaagaagtgatcacaatttcttcaggctcttgcatgaacaaaggtttttcctcttgttggatccattcttgatatacttttaccacttttctcatagctgctgcttcacaaattggtaataaaaatgcctgacgaaatatctctgtcacaaagtttacattactccttttagaagaaaaaactctgcgaactatttcaatgtctgtgagatgttcttcatcaatactacagagactagatgagctaggttctcgctccgtgagagtgcttgtattggaatgagactgttcgggttctgtagttctgtctgttttatcagcattatcatttttgctttcttctctggatactaaactagcagctgctctctgaatattctttggcaagacttcaccttccatcccaggaatatgaggtcctgtatgtggttttggctccagccagaaagaaaccagccaacgaatgacaataacacgagccttaatgaaaggctcctttgtacaatagattgcttcattggtttcagcatctttctttatcacgacataatgtggctttggtctcatctgcgggatgtcaagtataggatgatataaactgttttccttacagatgtttggaaaaatataaggcaagtaatatttcttaaaatgtgaaaacaaaaatgaaaatcccctttcttggttttctttgttcttccattctaaactttttacctgaatgactatgtattttagaagtgcttcaagaaaatagcttgtgagatcttcttgccctttatctcctgattgtggggggacaagaggagtgatttcttctatagtgacttgagtttcttgaaggttgagtggaggattaatgagattatctaaagttcgaggtccatgttcagactgtggtgctgaaaatccagggattaagcatgaaaacatccagagctgttctttgctacagttattctgaagagcttgcaaccatagtaagaaaagacgaacaccttcccgcctaatctttaaggagtttcctgtgtgaagtagcttctttaaaatcaatccaatactatgaaactgccatcgctgatgaattctttctggaagaagttgtaaaattttctcaaaaataaaaagtatagcatccaattcctctctttgagacttgtgacctttctgtttaagactagcttcaatagtcacaaaattttcaaagaacacatagtatatatgtgaaaaatgttggtcgaaaaactgtttaagatcaatagattctgcattctcgatgacgatgcgcaggtgcttgaggcgagtcagtgcgtccttcttggtgtctagcaccttctgggtggacttcttcacgtccccgtgcggcttcttggagaacatcctgtcgctgccactgccactgccactgccacagccggctcccagccgggtcccggcggcagaaagtggagggagtggacggggaggagactagccagagaggctcattagctccccagccttgcgggccagggcagagccgactccttcccgatccaggccagggccgccacct

SEQ ID NO: 10806 - RNA, 3579 nt, Homo sapiens
  source 1..3579: mol_type = other RNA
ctctagagggaagcactttctgaaccagtaatagttgcaacttcagcagagaaagcttgctgattaagactgcttgtttcagaatctatatgaagagtagttagactagccacttcctgctcttcagcactctgatgatggccagaacctgaatccacatcagcagaggacgtaaccccagtgtcggttccaaagccaaaattgtcaaattttcggccatcatattggaaagcgctgaaagaatccgaatgactatctgagctgataagatcactgctccctgcactggcaggagaagtccattctgagggcacacctgggtcatcaatagggcgcatctggttctgcttgtttagaatatcagggaggtctttgggaatttccaggctgcctggactacttcctcttcttgtcatagtcgaggcattaccacttcgaagtcgttctgctataaactcatccatcagatcaggaacattagcactgctgccgccaatatcactattaagaggaggcagtttttggctcatgtcctctttattgactttggctcgttcaacagtgaatggttccaagatgtcagaagtgctgctacttcgaggcaatggctgctcctcattcaaagcaccaaaaacttcatttccagtttcttcactttgtgaaaaatgtctgactctagttgagcggggaagtatttgagcatcatcaatatctgaaagctcatcagaaaggggagtgagaacaatatcaggcaagaagggtttggaagtatggatcagaacaggagcacttttagcactgcgtatataggccgatggcagagcacattcaccaatggatcggcttctcatggcgacagttttttgccgtactatactcctcgccttttcggttcctggagaaccagtggttgttgcactcctctgtctcattggggcttggccaggctgatcacgactccatcctctagaaaatgacttgtcaactgaaactttctgaaattcatgtccaactcctttccctttgtgctttttttgtttctgttcactcagcttatccaatggtaaatcactgagatccaaactatataaattcctagctaaaactttagttaatgtctccatagtcagtgaccactcagtggccaactcttcccaataggtcagcgatgacaatactgacagtaagtcatcccaaagttctcgggagatgtacacatttaggtttgctttgatccaggcaactataagggtctggaaaagtggtcctgcaagtcgacctgccaaggtcatattttttttcccttggaactgtagaaaagcttgtgatggcatcttcagtacagattccgtgactctgagcaacacaagcagcatctgttcccaagtctttttgtccattgatacttgtacaaccatgtaccgataaatgttaagaatgcgtttacacatatctgtgtgttcatccagaagattttttatttcatttgcaggttcaagaagaaatatatttgatgagtttataataaacacctgcaaaactgcctgggtaccagctcgtatgttttgttctgtggcttcttcagaggcgttatgaagagcaccttggtaggagccgttttttgcccaactggaatttcgaacatgatcagcagtattggtcccattttcctcttctcttttttctccttcttccattgaaatatcatggtctgtgacattttcaatgcaagggaggtctgaagaagtgatcacaatttcttcaggctcttgcatgaacaaaggtttttcctcttgttggatccattcttgatatacttttaccacttttctcatagctgctgcttcacaaattggtaataaaaatgcctgacgaaatatctctgtcacaaagtttacattactccttttagaagaaaaaactctgcgaactatttcaatgtctgtgagatgttcttcatcaatactacagagactagatgagctaggttctcgctccgtgagagtgcttgtattggaatgagactgttcgggttctgtagttctgtctgttttatcagcattatcatttttgctttcttctctggatactaaactagcagctgctctctgaatattctttggcaagacttcaccttccatcccaggaatatgaggtcctgtatgtggttttggctccagccagaaagaaaccagccaacgaatgacaataacacgagccttaatgaaaggctcctttgtacaatagattgcttcattggtttcagcatctttctttatcacgacataatgtggctttggtctcatctgcgggatgtcaagtataggatgatataaactgttttccttacagatgtttggaaaaatataaggcaagtaatatttcttaaaatgtgaaaacaaaaatgaaaatcccctttcttggttttctttgttcttccattctaaactttttacctgaatgactatgtattttagaagtgcttcaagaaaatagcttgtgagatcttcttgccctttatctcctgattgtggggggacaagaggagtgatttcttctatagtgacttgagtttcttgaaggttgagtggaggattaatgagattatctaaagttcgaggtccatgttcagactgtggtgctgaaaatccagggattaagcatgaaaacatccagagctgttctttgctacagttattctgaagagcttgcaaccatagtaagaaaagacgaacaccttcccgcctaatctttaaggagtttcctgtgtgaagtagcttctttaaaatcaatccaatactatgaaactgccatcgctgatgaattctttctggaagaagttgtaaaattttctcaaaaataaaaagtatagcatccaattcctctctttgagacttgtgacctttctgtttaagactagcttcaatagtcacaaaattttcaaagaacacatagtatatatgtgaaaaatgttggtcgaaaaactgtttaagatcaatagattctgcattctcgatgacgatgcgcaggtgcttgaggcgagtcagtgcgtccttcttggtgtctagcaccttctgggtggacttcttcacgtccccgtgcggcttcttggagaacatcctgtcgctgccactgccactgccactgccacagccggctcccagccgggtcccggcggcagaaagtggagggagtggacggggaggagactagccagagaggctcattagctccccagccttgcgggccagggcagagccgactccttcccgatccaggccagggccgccacctccacccgcctcgcgccgcggctccaaggcaccttcggccccagctccaatatggcggatccctctcccggccctgcacggagcgaggcagacccgggctggccgcctgccgccgccgctcgtctccagcggccgccgctcgccgccacaggccggggccccggacccagagccacgaaggtggagctctcggcggcaggagcacaactctctccctgaggcccccttaaggttgaagcttctttagcagcttacaccctgcagaggccgaaacggagacgagtgt

SEQ ID NO: 10807 - RNA, 1520 nt, Homo sapiens
  source 1..1520: mol_type = other RNA
ctctagagggaagcactttctgaaccagtaatagttgcaacttcagcagagaaagcttgctgattaagactgcttgtttcagaatctatatgaagagtagttagactagccacttcctgctcttcagcactctgatgatggccagaacctgaatccacatcagcagaggacgtaaccccagtgtcggttccaaagccaaaattgtcaaattttcggccatcatattggaaagcgctgaaagaatccgaatgactatctgagctgataagatcactgctccctgcactggcaggagaagtccattctgagggcacacctgggtcatcaatagggcgcatctggttctgcttgtttagaatatcagggaggtctttgggaatttccaggctgcctggactacttcctcttcttgtcatagtcgaggcattaccacttcgaagtcgttctgctataaactcatccatcagatcaggaacattagcactgctgccgccaatatcactattaagaggaggcagtttttggctcatgtcctctttattgactttggctcgttcaacagtgaatggttccaagatgtcagaagtgctgctacttcgaggcaatggctgctcctcattcaaagcaccaaaaacttcatttccagtttcttcactttgtgaaaaatgtctgactctagttgagcggggaagtatttgagcatcatcaatatctgaaagctcatcagaaaggggagtgagaacaatatcaggcaagaagggtttggaagtatggatcagaacaggagcacttttagcactgcgtatataggccgatggcagagcacattcaccaatggatcggcttctcatggctgaaattaacttgtatccttctcaagataaccaatttaacatggaagtcttcaattcagtcatccaaccttgaagcttgctcaagtctcagtctgaatcccagaagtgattatcagcaatttgcttcaagatcatcccacttttccagtgtgcttactgctcatcactccattttccactcatagttttattttggtcaaggaaatgagtaagaagagtcttagaggtttctctatttgcaaaccagtggtacgacgaaatgctagcaagaatatctaatagctccagaatatcaagttcactatgttgctggcaatacgagtcatgtaatgactttttaaaaagcccctttcttcccaattttttattaagaaaattttcaaatgtagaaaaaattaaaagatggtgaggcatggtggctcatgcctataatcccagcactttgggaggccgaggagggtggatcacttgaggtcaggagttcaagaccagcctggtcaacatggtgaaaccccttctcactaaaaatacaaaaattagctaggcgtggtggtgtgcgcctatagtcccagctactctacttgggaggctgaggcaggagaatcacttgaacccaggaggcggaggttgcagtgagctgagatcgcaccactgcactccagcctg

SEQ ID NO: 10808 - RNA, 3477 nt, Homo sapiens
  source 1..3477: mol_type = other RNA
ctctagagggaagcactttctgaaccagtaatagttgcaacttcagcagagaaagcttgctgattaagactgcttgtttcagaatctatatgaagagtagttagactagccacttcctgctcttcagcactctgatgatggccagaacctgaatccacatcagcagaggacgtaaccccagtgtcggttccaaagccaaaattgtcaaattttcggccatcatattggaaagcgctgaaagaatccgaatgactatctgagctgataagatcactgctccctgcactggcaggagaagtccattctgagggcacacctgggtcatcaatagggcgcatctggttctgcttgtttagaatatcagggaggtctttgggaatttccaggctgcctggactacttcctcttcttgtcatagtcgaggcattaccacttcgaagtcgttctgctataaactcatccatcagatcaggaacattagcactgctgccgccaatatcactgcagctttccttccaaaatagcccattacatgactgtacagatccctcagtggagcctctggtggcattctgttctgcctctttggctcgttcaacagtgaatggttccaagatgtcagaagtgctgctacttcgaggcaatggctgctcctcattcaaagcaccaaaaacttcatttccagtttcttcactttgtgaaaaatgtctgactctagttgagcggggaagtatttgagcatcatcaatatcgacagttttttgccgtactatactcctcgccttttcggttcctggagaaccagtggttgttgcactcctctgtctcattggggcttggccaggctgatcacgactccatcctctagaaaatgacttgtcaactgaaactttctgaaattcatgtccaactcctttccctttgtgctttttttgtttctgttcactcagcttatccaatggtaaatcactgagatccaaactatataaattcctagctaaaactttagttaatgtctccatagtcagtgaccactcagtggccaactcttcccaataggtcagcgatgacaatactgacagtaagtcatcccaaagttctcgggagatgtacacatttaggtttgctttgatccaggcaactataagggtctggaaaagtggtcctgcaagtcgacctgccaaggtcatattttttttcccttggaactgtagaaaagcttgtgatggcatcttcagtacagattccgtgactctgagcaacacaagcagcatctgttcccaagtctttttgtccattgatacttgtacaaccatgtaccgataaatgttaagaatgcgtttacacatatctgtgtgttcatccagaagattttttatttcatttgcaggttcaagaagaaatatatttgatgagtttataataaacacctgcaaaactgcctgggtaccagctcgtatgttttgttctgtggcttcttcagaggcgttatgaagagcaccttggtaggagccgttttttgcccaactggaatttcgaacatgatcagcagtattggtcccattttcctcttctcttttttctccttcttccattgaaatatcatggtctgtgacattttcaatgcaagggaggtctgaagaagtgatcacaatttcttcaggctcttgcatgaacaaaggtttttcctcttgttggatccattcttgatatacttttaccacttttctcatagctgctgcttcacaaattggtaataaaaatgcctgacgaaatatctctgtcacaaagtttacattactccttttagaagaaaaaactctgcgaactatttcaatgtctgtgagatgttcttcatcaatactacagagactagatgagctaggttctcgctccgtgagagtgcttgtattggaatgagactgttcgggttctgtagttctgtctgttttatcagcattatcatttttgctttcttctctggatactaaactagcagctgctctctgaatattctttggcaagacttcaccttccatcccaggaatatgaggtcctgtatgtggttttggctccagccagaaagaaaccagccaacgaatgacaataacacgagccttaatgaaaggctcctttgtacaatagattgcttcattggtttcagcatctttctttatcacgacataatgtggctttggtctcatctgcgggatgtcaagtataggatgatataaactgttttccttacagatgtttggaaaaatataaggcaagtaatatttcttaaaatgtgaaaacaaaaatgaaaatcccctttcttggttttctttgttcttccattctaaactttttacctgaatgactatgtattttagaagtgcttcaagaaaatagcttgtgagatcttcttgccctttatctcctgattgtggggggacaagaggagtgatttcttctatagtgacttgagtttcttgaaggttgagtggaggattaatgagattatctaaagttcgaggtccatgttcagactgtggtgctgaaaatccagggattaagcatgaaaacatccagagctgttctttgctacagttattctgaagagcttgcaaccatagtaagaaaagacgaacaccttcccgcctaatctttaaggagtttcctgtgtgaagtagcttctttaaaatcaatccaatactatgaaactgccatcgctgatgaattctttctggaagaagttgtaaaattttctcaaaaataaaaagtatagcatccaattcctctctttgagacttgtgacctttctgtttaagactagcttcaatagtcacaaaattttcaaagaacacatagtatatatgtgaaaaatgttggtcgaaaaactgtttaagatcaatagattctgcattctcgatgacgatgcgcaggtgcttgaggcgagtcagtgcgtccttcttggtgtctagcaccttctgggtggacttcttcacgtccccgtgcggcttcttggagaacatcctgtcgctgccactgccactgccactgccacagccggctcccagccgggtcccggcggcagaaagtggagggagtggacggggaggagactagccagagaggctcattagctccccagccttgcgggccagggcagagccgactccttcccgatccaggccagggccgccacctccacccgcctcgcgccgcggctccaaggcaccttcggccccagctccaatatggcggatccctctcccggccctgcacggagcgaggcagacccgggctggccgcctgccgccgccgctcgtctccagcggccgccgctcgccgccacaggccggggccccggacccagagccacgaaggtggagctctcggcggcaggagcacaactctctccctgaggcccccttaaggttgaagcttctttagcagcttacaccctgcagaggccgaaacggagacgagtgt

SEQ ID NO: 10809 - RNA, 1432 nt, Homo sapiens
  source 1..1432: mol_type = other RNA
ctctcaccactgccctcccacagcaagctctggacagagagtctcggcctggcctgcctgggtgggcttcactgacctccacagggatttgaattctcactgtcaatgctttcagctttctacctagaagaaatctgggggtgtggatgggggtaagagctgctgcttccttctaggtttagttggtcaggacccaggaaaaatatcagaaatgccagccactctttcctcttccagaatccttttctgaggccactgtttctctgggggtggctgagacactggctggagcaggtgctggtctcaggactaaaactctcagaatctggcaaccgccagattcaccaggaaagtgagtccagtcacagccattccttgaccttggggagtctaactcctgcctggggcagttcgcttgagtacccagaaagtggacggggcggcagaagcgagaatgggaacacccattcattcactggagcgctcactcatccatccacctaacccatcaaacacgcaggcaggcagagcttttcccaggcctctcccacccagatgtggaaagggagcaaagcctgacttctgacagcgacagctcctggaaagggcccagcacctgggggccctgcgttcccacgggagcccctgttcgaggccgtgcagccttcacagccgcagtcccgggccctgccgggtggaaggtggccccatcctctaccccgaccccactccacaggcaatgctggcagagaggtcctgggaggtgactgtttcccaagggcatcgatgtgagcaggggtcaggactgcatgctctgagtcccagcattctgggcctcagtttacccacatgtaaaacgagaggtcagagcagaagtgcaggcactggctaagcgctcacaccctggagcgcggctgtctacgtggaaatggccgtgaaggcaaaggacacatggaactgtggagagccagcgtgatggaaagactgaaacatctcactagtaatttgacactgatcccatgttgaaatcatcacgtgaaatacaatgttattgcaatgagtttcatctgcatctttttaatgtggccactagacaatgaaaagcacatcttcggctcatgctgtgtttctattggacggccctggcccagggcagcagttctcagccggctgtactttagcatcacctgcagagcccaaatactgtggtcatatcgtcatccatatttttaaaacttgactaacttgacggcagtccagaacttgaaccagtcagacttctggcctctctcgttctctctgtgcaaaccattctctctctctgtgcccgttgaatgaatggtaaaaatcagtttatctctttctataaagttttgattaataggaaaagggattcgtaaggctagtcttaagctgtagtaaatctggtgtg

SEQ ID NO: 10810 - RNA, 3783 nt, Homo sapiens
  source 1..3783: mol_type = other RNA
ctctcaccactgccctcccacagcaagctctggacagagagtctcggcctggcctgcctgggtgggcttcactgacctccacagggatttgaattctcactgtcaatgctttcagctttctacctagaagaaatctgggggtgtggatgggggtaagagctgctgcttccttctaggtttagttggtcaggacccaggaaaaatatcagaaatgccagccactctttcctcttccagaatccttttctgaggccactgtttctctgggggtggctgagacactggctggagcaggtgctggtctcaggactaaaactctcagaatctggcaaccgccagattcaccaggaaagtgagtccagtcacagccattccttgaccttggggagtctaactcctgcctggggcagttcgcttgagtacccagaaagtggacggggcggcagaagcgagaatgggaacacccattcattcactggagcgctcactcatccatccacctaacccatcaaacacgcaggcaggcagagcttttcccaggcctctcccacccagatgtggaaagggagcaaagcctgacttctgacagcgacagctcctggaaagggcccagcacctgggggccctgcgttcccacgggagcccctgttcgaggccgtgcagccttcacagccgcagtcccgggccctgccgggtggaaggtggccccatcctctaccccgaccccactccacaggcaatgctggcagagaggtcctgggaggtgactgtttcccaagggcatcgatgtgagcaggggtcaggactgcatgctctgagtcccagcattctgggcctcagtttacccacatgtaaaacgagaggtcagagcagaagtgcaggcactggctaagcgctcacaccctggagcgcggctgtctacgtggaaatggccgtgaaggcaaaggacacatggaactgtggagagccagcgtgatggaaagactgaaacatctcactagtaatttgacactgatcccatgttgaaatcatcacgtgaaatacaatgttattgcaatgagtttcatctgcatctttttaatgtggccactagacaatgaaaagcacatcttcggctcatgctgtgtttctattggacggccctggcccagggcagcagttctcagccggctgtactttagcatcacctgcagagcccaaatactgtggtcatatcgtcatccatatttttaaaacttgactaacttgacggcagtccagaacttgaacctgaattcattcttattggccaggtcttcacttcttgccagcagcacagcaggaggacaaagcagagggtcccgtctccttggctcactgctgtgctccctccagctgagggagaaggaccttataaaagtcttaagtgtcccagccttggtctccaggacagtgtggaatgtcaggacctgtgacatcatgaccaggaagggagctgctggcatcttgcctgggctgagcagagtttctatccagtctatgactgggtaggagggaggaggttggtgggagtcttaaggtaacagagatcctctctcccattgctttttatggtgacttcctccatcctgaggactctgaagactgaaggggtagacactaattagaactctaagtgccagtagccaaaagccaacaaaatctgctcccatggaaagaggtgtatttgaaggatgctggagaggtcattgagttacagagcaagtgccagaaccaacagatccagagggtctaatcacctcttaaaggccccttgaggaacagagccttgaagaacagaggcccgtggccccatgtccctttccactctctcccaccctcaaagttccagggtggtgaagaacaggagacagatgacccaggtttcagcatcctttccctcaaaccttctttctcagcatcagtcccaatctccccttggcagtgagactttcatcacaagaggagaacatggctgcatttccatgttatcatcctcccagcttgatttcctagactttctagagctttcttcatcagcacagtgacaaaccccaaaggagtcactctggttgacccccctggatcctatctcacccctggactgactcctatgtccagggctcagagtggggcacctggtttagactgggccaggagtggggtcccgggtgaacagccctcaaatctcagctccatggtagagagggagaaagaagtggtcctgaatgtacaaccgtgcctcctgagaccaggtcaggaccctaaggatggcttgaccaccagggatctttgaccctatttttttattgctgatatgggggtttgaaaagactttctcactttaaacattatttttcacctcggaattcttgtttgattcaatttcaattagctgggctttatgttttattattacattttcatttcccttaaaatgaatgcatggatattataatctgtgacttcactgtgtatcattctaacaatgaaatgattgggaatgatacacttggctcaggctgtcttttcctcagaatttcttaaaaataatattttattttttggagtagttttaagttaacagaaaaattgaacaaaaagtttccatatacctccttataaattttagagaaatactgaatgttgctgtggagaagtctgaggccaatgtgattaccgttctctgctgtgtgagatttactttgctgtttgaacacgtgaagtattatttccttatcttgaagttcaatagcataattaggatttatcttgatgtttttattccccattaagtttcacagaaaaaaaggtatgtttgatatgcaaatttaaacttttagtttcaagaacttctcttatcttaatctttgcatgtaccatcaggtatctgtttggttcttgactcagggacactggtttttcttatattggactttcattgtctgtcttcaatgtctaatagcttttcactgactaatgttactcctttgtctttttcacttctattcattttgtttttgtccatgcaagtcatttaatttctagaaatacctatattatttcttgtttctattctctattgtaatattgttagatcctcaatttaattatgcccctctatatcaattctattgtgttttgttcatctttgggcttttttgtaatgtgtcagtttttccatcccatgaagaattgagaggactttcctctgtcttttgtattgtgtttcctctgtgttgttgttttggttggccttttgcctggtattctttttctttgattgctattgttttaataagtttgtgctattccgtgtatttcttttcactttgcttgtatttgggcatgtctctcagatgttattatgatacacagtgaatgaccatttggtcctcttccaatcttctttaagtcatatttgttttctcctcacattcctgtaccctattctaagcaagagtttgaggactgggttgtgtaggctgcctcattttctatggcctaaagaaatggagttggggaaagagggtggaacaaagaaggtgcggtaataatgtcacattttttgaatttctaagttcatagaacaaatttctgctcccgaaaaacatgataagaaaaaatagaggtttcaaaccactgggaggagatgagatcattagaccgttcatctttatgtaaccagactcctcagttaaaggtcattttcaaagcacacctgcacttgtttttttcttatgaaaatatcctgtatatccttaa

SEQ ID NO: 10811 - RNA, 70 nt, Homo sapiens
  source 1..70: mol_type = other RNA
ctctctggccgtctaccttccacactgacaagggccgtggggacgtagctggccagacaggtgaccccag

SEQ ID NO: 10812 - RNA, 34 nt, Homo sapiens
  source 1..34: mol_type = other RNA
ctcttgagggaagcactttctgttcccaattgct

SEQ ID NO: 10813 - RNA, 2049 nt, Homo sapiens
  source 1..2049: mol_type = other RNA
ctgaagctcagagggctctgatgggatctgcagcagtgtggggggatgagacatcctcaggggcttcgtggagagagagggtctgagctagtggctgtcacatacaggctgttcatgttcactgtcatcattgtcaatacttccatatcatcaccaccaccatggttaacattgattgggttctgacaatgcgccaggcactattacattctttagatagctgattttgtttaaccttcatttctagctttacgaggttggtaccctgacccatcccctttataaatatcaaaaaacttacagaaaagtaactttaacttgttctaggtcacacagctcataattggttgagggagaaatggaaccaagtcatatgactaatgcttctcttttctaagctacttacgatccctactctcattgtttaactcctgaccatcctacaagttaccactcaatgtggacacagagcaacaaagcaagttatattttttaatctttttttttacctttaaactttttattttgaaatagttttagacatacagaggagttataaactcagcacagagttcctatatataccacattcagctatccctaatgttagcatcttataaatacacagcacaatggccaaaactatgaaaccaacattggtaacacactattaacaaaatgcagactttgttcagatctcgcaatttttccactgatgtcctttttctgttccaggacccaatctgggattccactttgcatactagttgactcattaggatctccttggtctcccatccatggcggttcttcagttttcacctgtctttcatgactttgacacttttgaagagtatctcatcatttcgtagaatgtcccttaatttggatttgtctcatgtttccccatggttagattgagggtatgcatcttgggaaagaatctacagtggtaacgtgccctctgtcatatcgggggcacatgatatctatgtgtcttgttactgatgatgttagtgttgatcacttggttaaggtggcgtctactggctttctctactgtactgttaacatgtttccctttgcgataataagtatttgcggggagaaactttgaaactatgcagcttaaatttccaaccactaacgttagcattcatcagtggatcttctctgtagcaattattactgtggttttctaatggtgatttttctattttcttcattcatactacaactattaattggaattagtctataaggaagagttgtttcttttcctccttttattttttggttcatttatttttaggagtatggactcatgggtatttactagattccttgtgttataatccaataccttcatttcatatttttgttcaaattcttcaatcttggccattaggagctctttcaggctgtctcctgtgtcctttctatatccccctgtcccctttttaaagcatttctttactttctggcaccaaaaggatgctccaggctgaggctttgacttagttcataaccagttgtctcttccttatcttctgtaagatgggtataagagattggcaggtttcctgaaacgtaagtgacagaatgtatgtcaaatacttgcaaagtgcctggcacatactaagtgctcaataaattagttgctattgtgaatgaagatgattctgttgttcaaaatcttgttggaactactttttgaagtcccttccaaactagtacattaaactattctaaagaatttagttgagtttgtttatagttaaaactcagggttttgttttgtttattttggtgctcagtggatctgaccccattgacccccttatttattagcccagtgcaaaatcattttggctccttccaaaaaccaatccatctccaatatcatgagtatttgcaattttttaagtgattccaaatgaggcctgtattcttgagagaacttctcaagtaaatgctataaaaatgttttgagtgcctgggcacagtagctcacacctgtaatcccagcactttgggaggccgacaggg

SEQ ID NO: 10814 - RNA, 2150 nt, Homo sapiens
  source 1..2150: mol_type = other RNA
ctgaagctcagagggctctgattcagaaagatcatcggatccgtctgagcttggctggtcggaagtctcatcatctgcttccttcgggttaaacacgtcggccaggtctgagtatgggtgtggcagtccgggtagcaggctcatgccgtgcctctctagggcaatgcatggcgggggcgggcggaagcagttcttcaggcagtagggagagtggaaggtgcagcggcctttgatccagtcgacttcgggggcgtggactcggagccagcggatgcctaggaccacagagaagttcggtgaaggtacgatgtcaaattcgatggactcctggtggttctggtggatacacaccaggggctccgtgtagagccagacaggctcgttgccaatcagcgagccgtccacggattggaccggctgtgggtacggcttctcgtagagctcgacgtagtgctcttgggcgaacttctcatccatgaagttgccgtcagctcccgaatccaccagggcctggaccgcgacgctgtggtaggggttcactctcaccatgagcagcaggaagaggtgggcgcgattgatgtccggatggacttcgctgggcaaccagctgctgaccatccacctctctggagcaggtgagtcgatccaggtcaggttccgggggcgggcctcggggggcagcctgagcatagctcttctctctgccagcttctcttctatttgcaggatgagcacaatcagactgtctagggaatccggctgagggacccggaatagatagtgcctgatctcctcgttgagcccctggcacaagtgggcctgcaggacttcatctggccagcccaagatgggtaccaggctctggaactcatcgatgtactcagtggcagagcggccgccctgcctgatggtgaacatggcctcttctgccacacgcagtgcctggcggtactcaaacacttcggacatggcctccaggaaggctgggaagtctccgatcagggggctgttttcctgcagtagagctttggcccattctaatgccaagccggacaggtgattgatgacatagccaactctcagacggtcgttatagaacattcttgggtagctctgtaaggtcagttggcagagtacgatgaactcgtggaattctctgcgatcgccagagaagtgctttggggcgggcagttggcctgcattgatccctttgatcaagatctcttctgctactctctgttgctctttgaggtcttgcattcggaagtacagcgagatgatggacctcaccatggccataagttctgcggttgagtgctcggtctggttttgctcttgaggagtctcctcccttcccgattccttcaggtcagtgtgagcctcttgttcttctcgggctcccgatgggttgactgatgcttctttcatcctatcagatgctccactgagtggatccccccttgcctggtgtgaaccgttgcatgactcctccaggtcttggagtaggtcattgggtggatcctctatttccttacgtgggccactggatggctcctccatgtcttggagtagatcagtgggcagctcttccatttcctggagtgggccactggggggctccttcttttcctgggctgggccgctggctggccctgcctctccccgcactccactgcccgacgtcgcctcggtggtgttggatgagccctcggaggactccatttgttttgatgatggattcttatgctccatcatcgtctcaaatgagtcttcagagggttctatcatttcgtcggatggaaaggagtgtattctgaagattggtaaggttgtgatggcgtccagtcagtagctgggaccgtggagatcagaaccttggctgcaagcgttcaagtggatctcctcccgtcctgtgccactcgatcctcgctgcttgcttccccgggcccagtcccaagcgtgaggctggggatgaagtgatgccggtggcttagtgatgccggtggcttcctgtcctcgaagctcagtcggtcgtctctcagctggtgtgaggctgggccaggatggaaccccagactctccgaggctccccaccacaccctgctgctgaaggctgctcagcgaggctgtgccgagtgctgggggggtgt

SEQ ID NO: 10815 - RNA, 290 nt, Homo sapiens
  source 1..290: mol_type = other RNA
ctgaagtgatgtgtaactgatcagtaggcaagttttacctacagctccgtctcccaccaccacacacttgatggcctgcatcagggccgctcgctgggccgcggcggcggcggcagggcgctgagataggaagcggcgggctcggggcgcggcggacgggcgcgcggcttgcgggcggcggggcgctgggtgccggggccgctgtccacgccgcctcgccctccgcggactggaagccgatgcccggcagcggccaccacccaaagctgaggaaaactgcagagaaacag

SEQ ID NO: 10816 - RNA, 2066 nt, Homo sapiens
  source 1..2066: mol_type = other RNA
ctgaatagctgggactacaggtaagtgccagcacatgtggctaatttttttacatctttgtagagatgaggtctcactattttaccaggctggtctcaaattcgtggcctattgtgatcctaccagctcaacctcccaaatcgctgggattgcagacatgagccactgtgcctgactcaaaaatcatactttattcttgagcccattggtcagggtagattcgcacactccctctgcagtgactccaggagcccctctcacagctcagagcggaagctgaggctgcagcctgccatcttctccgcatagtccgcatcgaagcgctcattctgcgccacggtgaaggtggtcttccagtccccagccatgcctttcctcatgaagggggagatgctgtggtccatgagctcctgggggacggtggtgtagttggtcatagggttcttcttcatctccttgaacgacgtgtgctgaaccatgaagtccatggtctcctctggcagggagcgccccacaaactccaggatcttttgaatctcccttttggggttctccttcatgtcttcatagaagaggtagagaacagggtgggtgcggctcagctcccaccactcctgcacgtgctggtaccaggacccgtaggacacttctccagccatgaacttttccaggaagctgtcccaggtcccaggctcagggtgcgccttttccatacggtggaaatggtagtaggagaccgccacgtcctttgggtttcgggcaacatagaccaccttgaccttctgatccaacagagtctgagggagcagagccaggggcaggtgtgacttgatgagccgtgggggcggtgtgtctttcagagtctccagccctgagggttcccctggatcattgacctcaaggaagggcacccgtacgtagatgggagcccggttacacttctctaggtcgccgccctggtagatcatgtccagtatctggctcacccaggtggtgccagacttggggtaggtgttgatgagcaggtcatcaggtcgggcttggaagctctgcaggggccccagtgcctctgcaaagtacttgatgagcgggacccccttcacgtactccagtggcgggcgggaggtgtcctggatcagctccatgttcctcttctaattctgagtcttctacttctttctcagtgtccatctggcacagccagatcaggtctccccaaagcagtgacttctcacagcaagggcattggccctctaggggcagaagctgccctggttcttcctgaagaaactcctctgccaggcagatcacatgggcccttagcaggcagccagggtgggggcaacacaagggcccctcttcatcctggatggtctgggcgcacagggagcagcaggcccctggatccccctggtctggctcaggctccgcgtcatcaaagggacctgcgcggcgccttggggccggggcctggggcggtggaggcccgaaggccagaggcacgtgcggcggcggcgggaggcagaggtcctggcggaggtctgggcgcacccagcgcagcgtgagcgggaggcgagcccagggcggtgcgcgcagcatgtgcgccagcacgcgcaggtggaaagcgaaggctgtctctcctcgcaggcgaggccccacgtgcgccaggcggcgcgaggcgtgcgggtgctgccaagcccactcaaaccgaagggcggccacggaggacgggaagccgtgcacgacgagcaccatctccctgaggaggagaaccgtgatgtccctgtcgcagcccagcgcctcagccgcgggtcccctccaatcccacccgagagcggggtcctcattcccggcttcagccgagaagtgcagccctctgcacctgcccacctcaggccctgcctccagcccaggtacccacctgtcccacctcctctctctcctgcattccacccgaccccagcgtgcccaccaagagccctatgctggaacccagcctggatcatcacccccgccccagctagctccttccctgagttccgccgcggagatgccccgggcaccgc

SEQ ID NO: 10817 - RNA, 2066 nt, Homo sapiens
  source 1..2066: mol_type = other RNA
ctgaatagctgggactacaggtaagtgccagcacatgtggctaatttttttacatctttgtagagatgaggtctcactattttaccaggctggtctcaaattcgtggcctattgtgatcctaccagctcaacctcccaaatcgctgggattgcagacatgagccactgtgcctgactcaaaaatcatactttattcttgagcccattggtcagggtagattcgcacactccctctgcagtgactccaggagcccctctcacagctcagagcggaagctgaggctgcagcctgccatcttctccgcatagtccgcatcgaagcgctcattctgcgccacggtgaaggtggtcttccagtccccagccatgcctttcctcatgaagggggagatgctgtggtccatgagctcctgggggacggtggtgtagttggtcatagggttcttcttcatctccttgaacgacgtgtgctgaaccatgaagtccatggtctcctctggcagggagcgccccacaaactccaggatcttttgaatctcccttttggggttctccttcatgtcttcatagaagaggtagagaacagggtgggtgcggctcagctcccaccactcctgcacgtgctggtaccaggacccgtaggacacttctccagccatgaacttttccaggaagctgtcccaggtcccaggctcagggtgcgccttttccatacggtggaaatggtagtaggagaccgccacgtcctttgggtttcgggcaacatagaccaccttgaccttctgatccaacagagtctgagggagcagagccaggggcaggtgtgacttgatgagccgtgggggcggtgtgtctttcagagtctccagccctgagggttcccctggatcattgacctcaaggaagggcacccgtacgtagatgggagcccggttacacttctctaggtcgccgccctggtagatcatgtccagtatctggctcacccaggtggtgccagacttggggtaggtgttgatgagcaggtcatcaggtcgggcttggaagctctgcaggggccccagtgcctctgcaaagtacttgatgagcgggacccccttcacgtactccagtggcgggcgggaggtgtcctggatcagctccatgttcctcttctaattctgagtcttctacttctttctcagtgtccatctggcacagccagatcaggtctccccaaagcagtgacttctcacagcaagggcattggccctctaggggcagaagctgccctggttcttcctgaagaaactcctctgccaggcagatcacatgggcccttagcaggcagccagggtgggggcaacacaagggcccctcttcatcctggatggtctgggcgcacagggagcagcaggcccctggatccccctggtctggctcaggctccgcgtcatcaaagggacctgcgcggcgccttggggccggggcctggggcggtggaggcccgaaggccagaggcacgtgcggcggcggcgggaggcagaggtcctggcggaggtctgggcgcacccagcgcagcgtgagcgggaggcgagcccagggcggtgcgcgcagcatgtgcgccagcacgcgcaggtggaaagcgaaggctgtctctcctcgcaggcgaggccccacgtgcgccaggcggcgcgaggcgtgcgggtgctgccaagcccactcaaaccgaagggcggccacggaggacgggaagccgtgcacgacgagcaccatctccctgaggaggagaacggtgatgtccctgtcgcagcccagcgcctcagccgcgggtcccctccaatcccacccgagagcggggtcctcattcccggcttcagccgagaagtgcagccctctgcacctgcccacctcaggccctgcctccagcccaggtacccacctgtcccacctcctctctctcctgcattccacccgaccccagcgtgcccaccaagagccctatgctggaacccagcctggatcatcacccccgccccagctagctccttccctgagttccgccgcggagatgccccgggcaccgc

SEQ ID NO: 10818 - RNA, 1222 nt, Homo sapiens
  source 1..1222: mol_type = other RNA
ctgaatagctgggactacaggtaagtgccagcacatgtggctaatttttttacatctttgtagagatgaggtctcactattttaccaggctggtctcaaattcgtggcctattgtgatcctaccagctcaacctcccaaatcgctgggattgcagacatgagccactgtgcctgactcaaaaatcatactttattcttgagcccattggtcagggtagattcgcacactccctctgcagtgactccaggagcccctctcacagctcagagcggaagctgaggctgcagcctgccatcttctccgcatagtccgcatcgaagcgctcattctgcgccacggtgaaggtggtcttccagtccccagccatgcctttcctcatgaagggggagatgctgtggtccatgagctcctgggggacggtggtgtagttggtcatagggttcttcttcatctccttgaacgacgtgtgctgaaccatgaagtccatggtctcctctggcagggagcgccccacaaactccaggatcttttgaatctcccttttggggttctccttcatgtcttcatagaagaggtagagaacagggtgggtgcggctcagctcccaccactcctgcacgtgctggtaccaggacccgtaggacacttctccagccatgaacttttccaggaagctgtcccaggtcccaggctcagggtgcgccttttccatacggtggaaatggtagtaggagaccgccacgtcctttgggtttcgggcaacatagaccaccttgaccttctgatccaacagagtctgagggagcagagccaggggcaggtgtgacttgatgagccgtgggggcggtgtgtctttcagagtctccagccctgagggttcccctggatcattgacctcaaggaagggcacccgtacgtagatgggagcccggttacacttctctaggtcgccgccctggtagatcatgtccagtatctggctcacccaggtggtgccagacttggggtaggtgttgatgagcaggtcatcaggtcgggcttggaagctctgcaggggccccagtgcctctgcaaagtacttgatgagcgggacccccttcacgtactccagtggcgggcgggaggtgtcctggatcagctccatgttcctgagctctcgggaacctgacctgttctctccttgcctgcaggggctgagtatgggtgtggtgtagggagtgt

SEQ ID NO: 10819 - RNA, 2043 nt, Homo sapiens
  source 1..2043: mol_type = other RNA
ctgaatagctgggactacaggtacaagccattgcgtctggctggaatattctttcatgtgaacccctagtagctattttagctttttaacatgacttaaagtgatccgtctaggaatcccattaagatctcctgcttactagttcctgccagtgccttccccagggtggacccggcgtctaaggtttcctgccccacctctaagaatctcactttatatcttgggccatccacagcctgggggctgggccctgttgtgtttgggaatggaccaacttttgttcttctgcttagggcctgcttgtctggactcctggttggcccttctgttctggttcccccatccttgacttggatggtgtttcccttaccagtttgtgacaataattgggctttccacggtttgactcaagtaactttatttttctctaaattattttatctggcaacatttctgtggctttaactattaactgtaaacataaaacagatgtgaggatgatcttattccaagaggtggccgctgtgttccagccccaggttgtctggtactttccttcctcactcctcacctcccacgtggcactatgcaaagcttcacattctatcttgttcttccttctccagtcgttcttgctcctcctgttccttctgcagccgggcctgtcttctcttttcagccaagatcttcgcagcctctcctgcatcagtggtgcctgctgtgggcttccccaaggctgcgctgttttcggctttccctcctgcggcagcagcatgcttctcgctggcatgcttgtccactacatgcttctctagggcttcctctccttgcgggccagcagcctgctgagccaaggtaccttccctttccttgttgctcttctctttctccgctttcctcttgggcatgtcttggccagaaagggcaggtaagcggtacttcacaggagaccctgggtagggaggtttcgttgtctttggagactgtggataagctttagtagctgtcttggatatcacaggagaagatggtctcttaggaatgcctccagaaaactcacatcttctcagaggggacccgaagttcacaacaggaagagaagttgctgttcgttgcccccgcttcaccttctccaccagagaggcctctcctcctgaaagggcttctttcccaacatctcctgcaccagatgtagacgtagatgtagctttcttcttctcaatgtttcgagtgggtgaagacttgtaagaagggttaagagggccaagaggagctaaacgaggacagacatggaatactgaatcattggcctgcccagagagcatgactgaagctctgcttctggctaaagaagactgtgtgggtgtcaacagtcgcgaaacaagaatggcttccattggactaaggtgcatgtgatgagctcggtctggggaataggatattgccacggtggatgaagacaggcgtttattcatgggaggctccgttggctttggcaaactcatagttgatgttgaaagtttgtcacatgcatcatgtcctccgggtccaatggccagtggtgctccccacgaatacttctttttcagctccagctgctgtgtgcgctccagggaccggcgcatcatcgcctccagccgttcctcctcctcccggagcttctgtttccttttctcttccacagcagctctcttttggtcctcccgctgccgctgctcttccagttttcgccatcgctcctccatttgcttttcgtactgcagcctggctcttttctgtttctccaggatctgttgctcccgagcagccagacatttttctctttcttctcgtctttctttggccaatctctgcctctcatctgatttcaaaaatccctccatgccttgaggccggtagttgggctgagaggtccgcaccgcgcccggttctgcgatcttccctgggagagaggttccccgcgcagtcccctcaggccgggatcccgtcccggagccgccgccgccgcgctccatcgggatgcgccggccgcacaggcgcact

SEQ ID NO: 10820 - RNA, 2142 nt, Homo sapiens
  source 1..2142: mol_type = other RNA
ctgaatagctgggactacaggtacaagccattgcgtctggctggaatattctttcatgtgaacccctagtagctattttagctttttaacatgacttaaagtgatccgtctaggaatcccattaagatctcctgcttactagttcctgccagtgccttccccagggtggacccggcgtctaaggtttcctgccccacctctaagaatctcactttatatcttgggccatccacagcctgggggctgggccctgttgtgtttgggaatggaccaacttttgttcttctgcttagggcctgcttgtctggactcctggttggcccttctgttctggttcccccatccttgacttggatggtgtttcccttaccagtttgtgacaataattgggctttccacggtttgactcaagtaactttatttttctctaaattattttatctggcaacatttctgtggctttaactattaactgtaaacataaaacagatgtgaggatgatcttattccaagaggtggccgctgtgttccagccccaggttgtctggtactttccttcctcactcctcacctcccacgtggcactatgcaaagcttcacattctatcttgttcttccttctccagtcgttcttgctcctcctgttccttctgcagccgggcctgtcttctcttttcagccaagatcttcgcagcctctcctgcatcagtggtgcctgctgtgggcttccccaaggctgcgctgttttcggctttccctcctgcggcagcagcatgcttctcgctggcatgcttgtccactacatgcttctctagggcttcctctccttgcgggccagcagcctgctgagccaaggtaccttccctttccttgttgctcttctctttctccgctttcctcttgggcatgtcttggccagaaagggcaggtaagcggtacttcacaggagaccctgggtagggaggtttcgttgtctttggagactgtggataagctttagtagctgtcttggatatcacaggagaagatggtctcttaggaatgcctccagaaaactcacatcttctcagaggggacccgaagttcacaacaggaagagaagttgctgttcgttgcccccgcttcaccttctccaccagagaggcctctcctcctgaaagggcttctttcccaacatctcctgcaccagatgtagacgtagatgtagctttcttcttctcaatgtttcgagtgggtgaagacttgtaagaagggttaagagggccaagaggagctaaacgaggacagacatggaatactgaatcattggcctgcccagagagcatgactgaagctctgcttctggctaaagaagactgtgtgggtgtcaacagtcgcgaaacaagaatggcttccattggactaaggtgcatgtgatgagctcggtctggggaataggatattgccacggtggatgaagacaggcgtttattcatgggaggctccgttggctttggcaaactcatagttgatgttgaaagtttgtcacatgcgttggtggactcggcagctgcggcagtggtccctgcatccggagggagggtgctggctgctaaacctagaggagggggtggggtattttctgattcaccatcatgtcctccgggtccaatggccagtggtgctccccacgaatacttctttttcagctccagctgctgtgtgcgctccagggaccggcgcatcatcgcctccagccgttcctcctcctcccggagcttctgtttccttttctcttccacagcagctctcttttggtcctcccgctgccgctgctcttccagttttcgccatcgctcctccatttgcttttcgtactgcagcctggctcttttctgtttctccaggatctgttgctcccgagcagccagacatttttctctttcttctcgtctttctttggccaatctctgcctctcatctgatttcaaaaatccctccatgccttgaggccggtagttgggctgagaggtccgcaccgcgcccggttctgcgatcttccctgggagagaggttccccgcgcagtcccctcaggccgggatcccgtcccggagccgccgccgccgcgctccatcgggatgcgccggccgcacaggcgcact

SEQ ID NO: 10821 - RNA, 1896 nt, Homo sapiens
  source 1..1896: mol_type = other RNA
ctgaatagctgggactacaggtacaagccattgcgtctggctggaatattctttcatgtgaacccctagtagctattttagctttttaacatgacttaaagtgatccgtctaggaatcccattaagatctcctgcttactagttcctgccagtgccttccccagggtggacccggcgtctaaggtttcctgccccacctctaagaatctcactttatatcttgggccatccacagcctgggggctgggccctgttgtgtttgggaatggaccaacttttgttcttctgcttagggcctgcttgtctggactcctggttggcccttctgttctggttcccccatccttgacttggatggtgtttcccttaccagtttgtgacaataattgggctttccacggtttgactcaagtaactttatttttctctaaattattttatctggcaacatttctgtggctttaactattaactgtaaacataaaacagatgtgaggatgatcttattccaagaggtggccgctgtgttccagccccaggttgtctggtactttccttcctcactcctcacctcccacgtggcactatgcaaagcttcacattctatcttgttcttccttctccagtcgttcttgctcctcctgttccttctgcagccgggcctgtcttctcttttcagccaagatcttcgcagcctctcctgcatcagtggtgcctgctgtgggcttccccaaggctgcgctgttttcggctttccctcctgcggcagcagcatgcttctcgctggcatgcttgtccactacatgcttctctagggcttcctctccttgcgggccagcagcctgctgagccaaggtaccttccctttccttgttgctcttctctttctccgctttcctcttgggcatgtcttggccagaaagggcaggtaagcggtacttcacaggagaccctgggtagggaggtttcgttgtctttggagactgtggataagctttagtagctgtcttggatatcacaggagaagatggtctcttaggaatgcctccagaaaactcacatcttctcagaggggacccgaagttcacaacaggaagagaagttgctgttcgttgcccccgcttcaccttctccaccagagaggcctctcctcctgaaagggcttctttcccaacatctcctgcaccagatgtagacgtagatgtagctttcttcttctcaatgtttcgagtgggtgaagacttgtaagaagggttaagagggccaagaggagctcggtctggggaataggatattgccacggtggatgaagacaggcgtttattcatgggaggctccgttggctttggcaaactcatagttgatgttgaaagtttgtcacatgcatcatgtcctccgggtccaatggccagtggtgctccccacgaatacttctttttcagctccagctgctgtgtgcgctccagggaccggcgcatcatcgcctccagccgttcctcctcctcccggagcttctgtttccttttctcttccacagcagctctcttttggtcctcccgctgccgctgctcttccagttttcgccatcgctcctccatttgcttttcgtactgcagcctggctcttttctgtttctccaggatctgttgctcccgagcagccagacatttttctctttcttctcgtctttctttggccaatctctgcctctcatctgatttcaaaaatccctccatgccttgaggccggtagttgggctgagaggtccgcaccgcgcccggttctgcgatcttccctgggagagaggttccccgcgcagtcccctcaggccgggatcccgtcccggagccgccgccgccgcgctccatcgggatgcgccggccgcacaggcgcact

SEQ ID NO: 10822 - RNA, 5804 nt, Homo sapiens
  source 1..5804: mol_type = other RNA
ctgaatagctgggactacaggtacacaccaccacacccagctaatttttgtatttttagtagagacagggtttcaccatgttggccaggatggtctccatctaccgacctcaagatctgcccatctcggcctcctgaagtgctgggattacaggcaattttttttttttaataaaatggaatttaagcctgtaatgtctttttaaggaatcaaaagtggtcatgtgataaatatgatacatagatacataatatatattttttccagttttaagaagttttgttaagaaggttttaaaaatattttaaatgcaacaagtttaaagataataaaagccacaagtattctagttatatgagattattctttagtcaaacaaaaccatctatattataaatcttgtgaaacaacttgagtatcaaagtacttccagtatgcattaatttaataagtttcaaagtcagaattctagtccaactgaaatatctgtagtcacattatcaggcttttcatagcttcacacttttaaacaacattttaaaagttaaatcaacataatatatccaaaaattcaaccaatatctatttacaaacatttacttaaaactaattttcatcaaatcaattgtggtttttgttggtttgttttttgagacagagtttcgctctttgttgcccaggctggagtgcagtggtgcgatcttggctcactggaacctctgcctcccaggttcaagggattctcctgcctcagcttcccaagtaactgggattacaggtgcccgccaccatgcctggctaatttttgtatttttagtggagacagggttttaccatgctggccaggctggtcatgaactcctgacctcaggtgatccacctgccttggcctgccaaagtgctgagattacaggtgtgagccaccgtgcccggccaaataaattgtgttttaaataaagttaacataaattgactagagtatactgtgtaaattattgtacacattaatcaaaactaatatccatgcatgctgaatctcttaaaatagtcactttatcacctaatgcaagttttcatatatatattcgactgcattttgtgatttttacccgccaatttttttcaagcctatataacttacacctttacaatgggacagttaaacttcagataaaaaaactggtaacattttcttttttttaaaagtattttgaatgtgtatccatttattaatatttactaaacttataactgaaaacttttattaaaacagctaacgttagtggtttactatgcattttataaaggagaacgtaagtgtttgttaagttgaagatcactgtgcacaccttacatttcaacatttcaagatattcaatcattcaaatatccattaagtacttactgtatgtctagcactattctaggtgttgcacaatttaatatgtttcaatatttcaaccatatgatattttggtatcttttatgctgtgtgaaacttttatatgctttttagattattcagtcctttataatttaaatgtttcctccttcccaaacgtagctattactgtttataaaggaggcacctatttttcctttaaattatatatatatatatattttgaagttaatgactaaaattcactgctatttcccacctctcccaacctgcaatccttctcccaacctctggcacttgagcaacaaagattaaggtaatgctaacccatgaaagtttttctttaaaaaaaaaaatcaagcatggacaaaaatcttctatcagaatggattgagtcgtattccagtccctaaaggtgagaatggattcacctttgcccacatcaaagcatcattcaaggagatagcagatttcccgtcttcaaggaaaaacacagggccctggatttttaatcccgtaagacaagaaatgtgaatatcagaatgacttggaagatttgatccagtcacataatctggtccaataattcctttcagtgactcttcttttagtctctttaataaagttgcataaatcattctttgtgaatcagaagggggtgtatacggagagtcttctaatgatctgttggtggactgtgtgcaagctctccatgcatccaattcctcagaaagatattcaatttttaaaggtactgacacctcccgacgttttaatagctgacttgtgtactcataaagtgctggaacaatgctttggtactgtcttctgatagccagtaatgcaccaatgtaaccacataatatcagcaactcatttcgagcttcagtacacgtatgcaagagtaatttttcagtacgaatatagctcagtaggtcaagaacagggtatatggtatccaaagtccagtctgagctactgatgtattctttaacaaagctaataccaataggaagggctttttcaggttcttgacttaacaagtaatattttacagtttcaaatatattgtcatctgcacgggctgtctcagctaactgcatacattcttccactgtgggtagcttacacttatcatgaaggtcatttatctcttcagtacatcctgggtagaaagcacagagttttattaaatgtagttcattatcaggaatcatcagaagaagatcagctgccaaattccatactgaaatcatcatgcactttctcgccagtaattctaaggcatagtgggttgctggtgctgcagactctcctagtactgtgcccacacagactgccaactccagttcatttccgcgaatcaggtatgccatagcaagctcaatattatctatggcaagatggcaacatgcggctagtactgctcgaccatcttgaaaataccattctgccagttctttactgactttgtgcaggagttcattaaagtcttccttgtagatatcatcagaatatgaagctcctttaggcacggaaacatgtaagggctgcatatttccttcacaagcagcctgtgcaacaagcagagcttctttaagctgacctcttgacatgaaaaaatggactagctttttcacatcaccaatggctatgcagtatggaatgacatcatccttatcttcctggattaattggtcagctctcctctgcattaacttcttccagtatttcacagagactcctggtgcaattgacagggctttgtcccactctccaagttcaaccataagttcacagtatctctgaatttgtcctaatctcaagtggatttcagcagcttccttcagtctttcctctttagcaggtacaccaataccaccaccaaatttagacatcttgactgttgttagttcttgagcttcagatgttctaaatttaatcagatgtttcaagtgcattattcctttgcagtagttctgaggaagtaagctatcatcctgtccttttatcacagcaaccaagttccataaattgtcactgccacctggaggagataaacattctgagaaccatcttagttttttcacttgagaattagcagttagtttttctatttcctgtctaatatctcttgacactttaccacacagtagaggaggagtgcctggttctatagcataatcagtgttcccaataatttcttcccaagatctgtctgccagaatatttatttgtacaggagtgactaaggctgttaatgaccagagtctcactgtagagtcacgggagcaagaggccatagtgaaggggcgactgggatggcaggttaaaccatatacatctgcaccgtgatcatacacagtatccacacaagttccttctcgagtgtcccatacttttatagtatagtcccagctgccagatatgagcagatatggaatctcagtattccacattaatcctctcacaggtgcagtgtgtccattaagaatattgatgcaagcatcctgagtataatcccagattcgaacggtaccatcatcagaaccactgcaaagaattccctctctcagaggagaccatttaacatgaaacacttttgctgtatgcccactaaatactttcaatggttgatctgagctggtggctacataataaacacgaacatttgtgtcttcacagccagtggctatcatgtctttattgttttggctccaatcacaaccaaacactgcagctggatgtttatatttgtgtagcactttaccatcaattgttcgaataatacagaaaccatcactgctgcaggttgctattcttttagaatctttatgactccaggcaatgcagaatattccatttgttccatgctcattaaatcgttgtataattttgcccttttgaacattccaaataaaagcaccatttcgggaagttcccccagcaatacaatttaaaccacctggagcccaagaaagggaataaataacaccttcattacccggggatgtgtacactgctgttaatgtgtttatatcccagacttttatagtgccatcaaatgaagctgttgctaaaagattaggatcgtcaggtttgaatttgcagtcaaagatagtttccacatgtcccaagtctctaagaaaatcccacttcttagctcccatatcataaagtccaactccaccatccaagaaacaacacactgcatgaccaggaggaagagaaaatgcttgattctgtgttaaagttgggggtggaactgcttcgcttgttgaggatgtataatgatttttggttggagattggactgaaaacttttttcttggaggagaattaagtacatgtaagcagtgaaatcctgttttctttaatttaagattatcaataggtgttgttcttgaaacattccaaatgcgtaaaacacccacttgagaatagttctgcatggctgaggaggcctcaggaaacttacaatcatggtggaaggcaaagtagaagcaggcaccttctccagttataaacatcccaggagcactgggaacccaggctaagcactgtacagaagctgctgcactgggaagattaaatgttgttatgcaagaaagtgattcagaatctaccaggcgaattccataatgcaaattaaccactagaagataatcagtagatagtgggtcccattccaaggccgtaactggatcctcttcatctgtcccttcaagagattctggtctcaaaacatgtttctgatttttattacctggatgaaaaattgatagacttccatcaatatgaccaaacacaactttccccttttggtgtgtatgccatctgaacatacagatatcagacaagaagctatgagcatctttgtgtacaatcactccactatctggtcctgagatggtccaaatgaacagtgggcctctgtgggaaacaaatgccaccacatcctctgcattccagcaccaactaagagaagcagggatcccttttgtactgtcgagtttagcaatgactttttgttctgcaacattccaaatgatcactaaattatcagtactgccacttgcaaacagatcaggattatgtggacaccaagaaattgctgtgattgtttttttatgttcagacataattgcgtgaagtttgaattcattataacggtgatccaactgataaatatagatagccagggtcgcacaatatgcaaacctgtctccactggcagcacatacatccttgttccatggctgacatccagcagccagcaatcccacttgccttacctgggacatgtttgcctggaggaggaggcggctgcagcggcggacagcggaaggtgctgaagccggcgggcgcagctgcgaggcgagcaccaccaacgcgcggaccc

SEQ ID NO: 10823 - RNA, 5879 nt, Homo sapiens
  source 1..5879: mol_type = other RNA
ctgaatagctgggactacaggtacacaccaccacacccagctaatttttgtatttttagtagagacagggtttcaccatgttggccaggatggtctccatctaccgacctcaagatctgcccatctcggcctcctgaagtgctgggattacaggcaattttttttttttaataaaatggaatttaagcctgtaatgtctttttaaggaatcaaaagtggtcatgtgataaatatgatacatagatacataatatatattttttccagttttaagaagttttgttaagaaggttttaaaaatattttaaatgcaacaagtttaaagataataaaagccacaagtattctagttatatgagattattctttagtcaaacaaaaccatctatattataaatcttgtgaaacaacttgagtatcaaagtacttccagtatgcattaatttaataagtttcaaagtcagaattctagtccaactgaaatatctgtagtcacattatcaggcttttcatagcttcacacttttaaacaacattttaaaagttaaatcaacataatatatccaaaaattcaaccaatatctatttacaaacatttacttaaaactaattttcatcaaatcaattgtggtttttgttggtttgttttttgagacagagtttcgctctttgttgcccaggctggagtgcagtggtgcgatcttggctcactggaacctctgcctcccaggttcaagggattctcctgcctcagcttcccaagtaactgggattacaggtgcccgccaccatgcctggctaatttttgtatttttagtggagacagggttttaccatgctggccaggctggtcatgaactcctgacctcaggtgatccacctgccttggcctgccaaagtgctgagattacaggtgtgagccaccgtgcccggccaaataaattgtgttttaaataaagttaacataaattgactagagtatactgtgtaaattattgtacacattaatcaaaactaatatccatgcatgctgaatctcttaaaatagtcactttatcacctaatgcaagttttcatatatatattcgactgcattttgtgatttttacccgccaatttttttcaagcctatataacttacacctttacaatgggacagttaaacttcagataaaaaaactggtaacattttcttttttttaaaagtattttgaatgtgtatccatttattaatatttactaaacttataactgaaaacttttattaaaacagctaacgttagtggtttactatgcattttataaaggagaacgtaagtgtttgttaagttgaagatcactgtgcacaccttacatttcaacatttcaagatattcaatcattcaaatatccattaagtacttactgtatgtctagcactattctaggtgttgcacaatttaatatgtttcaatatttcaaccatatgatattttggtatcttttatgctgtgtgaaacttttatatgctttttagattattcagtcctttataatttaaatgtttcctccttcccaaacgtagctattactgtttataaaggaggcacctatttttcctttaaattatatatatatatatattttgaagttaatgactaaaattcactgctatttcccacctctcccaacctgcaatccttctcccaacctctggcacttgagcaacaaagattaaggtaatgctaacccatgaaagtttttctttaaaaaaaaaaatcaagcatggacaaaaatcttctatcagaatggattgagtcgtattccagtccctaaaggtgagaatggattcacctttgcccacatcaaagcatcattcaaggagatagcagatttcccgtcttcaaggaaaaacacagggccctggatttttaatcccgtaagacaagaaatgtgaatatcagaatgacttggaagatttgatccagtcacataatctggtccaataattcctttcagtgactcttcttttagtctctttaataaagttgcataaatcattctttgtgaatcagaagggggtgtatacggagagtcttctaatgatctgttggtggactgtgtgcaagctctccatgcatccaattcctcagaaagatattcaatttttaaaggtactgacacctcccgacgttttaatagctgacttgtgtactcataaagtgctggaacaatgctttggtactgtcttctgatagccagtaatgcaccaatgtaaccacataatatcagcaactcatttcgagcttcagtacacgtatgcaagagtaatttttcagtacgaatatagctcagtaggtcaagaacagggtatatggtatccaaagtccagtctgagctactgatgtattctttaacaaagctaataccaataggaagggctttttcaggttcttgacttaacaagtaatattttacagtttcaaatatattgtcatctgcacgggctgtctcagctaactgcatacattcttccactgtgggtagcttacacttatcatgaaggtcatttatctcttcagtacatcctgggtagaaagcacagagttttattaaatgtagttcattatcaggaatcatcagaagaagatcagctgccaaattccatactgaaatcatcatgcactttctcgccagtaattctaaggcatagtgggttgctggtgctgcagactctcctagtactgtgcccacacagactgccaactccagttcatttccgcgaatcaggtatgccatagcaagctcaatattatctatggcaagatggcaacatgcggctagtactgctcgaccatcttgaaaataccattctgccagttctttactgactttgtgcaggagttcattaaagtcttccttgtagatatcatcagaatatgaagctcctttaggcacggaaacatgtaagggctgcatatttccttcacaagcagcctgtgcaacaagcagagcttctttaagctgacctcttgacatgaaaaaatggactagctttttcacatcaccaatggctatgcagtatggaatgacatcatccttatcttcctggattaattggtcagctctcctctgcattaacttcttccagtatttcacagagactcctggtgcaattgacagggctttgtcccactctccaagttcaaccataagttcacagtatctctgaatttgtcctaatctcaagtggatttcagcagcttccttcagtctttcctctttagcaggtacaccaataccaccaccaaatttagacatcttgactgttgttagttcttgagcttcagatgttctaaatttaatcagatgtttcaagtgcattattcctttgcagtagttctgaggaagtaagctatcatcctgtccttttatcacagcaaccaagttccataaattgtcactgccacctggaggagataaacattctgagaaccatcttagttttttcacttgagaattagcagttagtttttctatttcctgtctaatatctcttgacactttaccacacagtagaggaggagtgcctggttctatagcataatcagtgttcccaataatttcttcccaagatctgtctgccagaatatttatttgtacaggagtgactaaggctgttaatgaccagagtctcactgtagagtcacgggagcaagaggccatagtgaaggggcgactgggatggcaggttaaaccatatacatctgcaccgtgatcatacacagtatccacacaagttccttctcgagtgtcccatacttttatagtatagtcccagctgccagatatgagcagatatggaatctcagtattccacattaatcctctcacaggtgcagtgtgtccattaagaatattgatgcaagcatcctgagtataatcccagattcgaacggtaccatcatcagaaccactgcaaagaattccctctctcagaggagaccatttaacatgaaacacttttgctgtatgcccactaaatactttcaatggttgatctgagctggtggctacataataaacacgaacatttgtgtcttcacagccagtggctatcatgtctttattgttttggctccaatcacaaccaaacactgcagctggatgtttatatttgtgtagcactttaccatcaattgttcgaataatacagaaaccatcactgctgcaggttgctattcttttagaatctttatgactccaggcaatgcagaatattccatttgttccatgctcattaaatcgttgtataattttgcccttttgaacattccaaataaaagcaccatttcgggaagttcccccagcaatacaatttaaaccacctggagcccaagaaagggaataaataacaccttcattacccggggatgtgtacactgctgttaatgtgtttatatcccagacttttatagtgccatcaaatgaagctgttgctaaaagattaggatcgtcaggtttgaatttgcagtcaaagatagtttccacatgtcccaagtctctaagaaaatcccacttcttagctcccatatcataaagtccaactccaccatccaagaaacaacacactgcatgaccaggaggaagagaaaatgcttgattctgtgttaaagttgggggtggaactgcttcgcttgttgaggatgtataatgatttttggttggagattggactgaaaacttttttcttggaggagaattaagtacatgtaagcagtgaaatcctgttttctttaatttaagattatcaataggtgttgttcttgaaacattccaaatgcgtaaaacacccacttgagaatctccagttataaacatcccaggagcactgggaacccaggctaagcactgtacagaagctgctgcactgggaagattaaatgttgttatgcaagaaagtgattcagaatctaccaggcgaattccataatgcaaattaaccactagaagataatcagtagatagtgggtcccattccaaggccgtaactggatcctcttcatctgtcccttcaagagattctggtctcaaaacatgtttctgatttttattacctggatgaaaaattgatagacttccatcaatatgaccaaacacaactttccccttttggtgtgtatgccatctgaacatacagatatcagacaagaagctatgagcatctttgtgtacaatcactccactatctggtcctgagatggtccaaatgaacagtgggcctctgtgggaaacaaatgccaccacatcctctgcattccagcaccaactaagagaagcagggatcccttttgtactgtcgagtttagcaatgactttttgttctgcaacattccaaatgatcactaaattatcagtactgccacttgcaaacagatcaggattatgtggacaccaagaaattgctgtgattgtttttttatgttcagacataattgcgtgaagtttgaattcattataacggtgatccaactgataaatatagatagccagggtcgcacaatatgcaaacctgtctccactggcagcacatacatccttgttccatggctgacatccagcagccagcaatcccacttgccttacctgggacatgtttgcctggaggaggaggcggctgcagcggcggacagcggaaggtgctgaagccggcgggcgcagctgcgaggcgagcaccaccaacgcgcggaccctccccgccctccccgcctgctcgctcagggcgcccgggggcggggcggccgggcccgcgggctccgaggggcgggaagcgtgctccgcaagccccagcgcggagccacgatggaaggcgccgcgagcccgatctccagggtctgccc

SEQ ID NO: 10824 - RNA, 5861 nt, Homo sapiens
  source 1..5861: mol_type = other RNA
ctgaatagctgggactacaggtacacaccaccacacccagctaatttttgtatttttagtagagacagggtttcaccatgttggccaggatggtctccatctaccgacctcaagatctgcccatctcggcctcctgaagtgctgggattacaggcaattttttttttttaataaaatggaatttaagcctgtaatgtctttttaaggaatcaaaagtggtcatgtgataaatatgatacatagatacataatatatattttttccagttttaagaagttttgttaagaaggttttaaaaatattttaaatgcaacaagtttaaagataataaaagccacaagtattctagttatatgagattattctttagtcaaacaaaaccatctatattataaatcttgtgaaacaacttgagtatcaaagtacttccagtatgcattaatttaataagtttcaaagtcagaattctagtccaactgaaatatctgtagtcacattatcaggcttttcatagcttcacacttttaaacaacattttaaaagttaaatcaacataatatatccaaaaattcaaccaatatctatttacaaacatttacttaaaactaattttcatcaaatcaattgtggtttttgttggtttgttttttgagacagagtttcgctctttgttgcccaggctggagtgcagtggtgcgatcttggctcactggaacctctgcctcccaggttcaagggattctcctgcctcagcttcccaagtaactgggattacaggtgcccgccaccatgcctggctaatttttgtatttttagtggagacagggttttaccatgctggccaggctggtcatgaactcctgacctcaggtgatccacctgccttggcctgccaaagtgctgagattacaggtgtgagccaccgtgcccggccaaataaattgtgttttaaataaagttaacataaattgactagagtatactgtgtaaattattgtacacattaatcaaaactaatatccatgcatgctgaatctcttaaaatagtcactttatcacctaatgcaagttttcatatatatattcgactgcattttgtgatttttacccgccaatttttttcaagcctatataacttacacctttacaatgggacagttaaacttcagataaaaaaactggtaacattttcttttttttaaaagtattttgaatgtgtatccatttattaatatttactaaacttataactgaaaacttttattaaaacagctaacgttagtggtttactatgcattttataaaggagaacgtaagtgtttgttaagttgaagatcactgtgcacaccttacatttcaacatttcaagatattcaatcattcaaatatccattaagtacttactgtatgtctagcactattctaggtgttgcacaatttaatatgtttcaatatttcaaccatatgatattttggtatcttttatgctgtgtgaaacttttatatgctttttagattattcagtcctttataatttaaatgtttcctccttcccaaacgtagctattactgtttataaaggaggcacctatttttcctttaaattatatatatatatatattttgaagttaatgactaaaattcactgctatttcccacctctcccaacctgcaatccttctcccaacctctggcacttgagcaacaaagattaaggtaatgctaacccatgaaagtttttctttaaaaaaaaaaatcaagcatggacaaaaatcttctatcagaatggattgagtcgtattccagtccctaaaggtgagaatggattcacctttgcccacatcaaagcatcattcaaggagatagcagatttcccgtcttcaaggaaaaacacagggccctggatttttaatcccgtaagacaagaaatgtgaatatcagaatgacttggaagatttgatccagtcacataatctggtccaataattcctttcagtgactcttcttttagtctctttaataaagttgcataaatcattctttgtgaatcagaagggggtgtatacggagagtcttctaatgatctgttggtggactgtgtgcaagctctccatgcatccaattcctcagaaagatattcaatttttaaaggtactgacacctcccgacgttttaatagctgacttgtgtactcataaagtgctggaacaatgctttggtactgtcttctgatagccagtaatgcaccaatgtaaccacataatatcagcaactcatttcgagcttcagtacacgtatgcaagagtaatttttcagtacgaatatagctcagtaggtcaagaacagggtatatggtatccaaagtccagtctgagctactgatgtattctttaacaaagctaataccaataggaagggctttttcaggttcttgacttaacaagtaatattttacagtttcaaatatattgtcatctgcacgggctgtctcagctaactgcatacattcttccactgtgggtagcttacacttatcatgaaggtcatttatctcttcagtacatcctgggtagaaagcacagagttttattaaatgtagttcattatcaggaatcatcagaagaagatcagctgccaaattccatactgaaatcatcatgcactttctcgccagtaattctaaggcatagtgggttgctggtgctgcagactctcctagtactgtgcccacacagactgccaactccagttcatttccgcgaatcaggtatgccatagcaagctcaatattatctatggcaagatggcaacatgcggctagtactgctcgaccatcttgaaaataccattctgccagttctttactgactttgtgcaggagttcattaaagtcttccttgtagatatcatcagaatatgaagctcctttaggcacggaaacatgtaagggctgcatatttccttcacaagcagcctgtgcaacaagcagagcttctttaagctgacctcttgacatgaaaaaatggactagctttttcacatcaccaatggctatgcagtatggaatgacatcatccttatcttcctggattaattggtcagctctcctctgcattaacttcttccagtatttcacagagactcctggtgcaattgacagggctttgtcccactctccaagttcaaccataagttcacagtatctctgaatttgtcctaatctcaagtggatttcagcagcttccttcagtctttcctctttagcaggtacaccaataccaccaccaaatttagacatcttgactgttgttagttcttgagcttcagatgttctaaatttaatcagatgtttcaagtgcattattcctttgcagtagttctgaggaagtaagctatcatcctgtccttttatcacagcaaccaagttccataaattgtcactgccacctggaggagataaacattctgagaaccatcttagttttttcacttgagaattagcagttagtttttctatttcctgtctaatatctcttgacactttaccacacagtagaggaggagtgcctggttctatagcataatcagtgttcccaataatttcttcccaagatctgtctgccagaatatttatttgtacaggagtgactaaggctgttaatgaccagagtctcactgtagagtcacgggagcaagaggccatagtgaaggggcgactgggatggcaggttaaaccatatacatctgcaccgtgatcatacacagtatccacacaagttccttctcgagtgtcccatacttttatagtatagtcccagctgccagatatgagcagatatggaatctcagtattccacattaatcctctcacaggtgcagtgtgtccattaagaatattgatgcaagcatcctgagtataatcccagattcgaacggtaccatcatcagaaccactgcaaagaattccctctctcagaggagaccatttaacatgaaacacttttgctgtatgcccactaaatactttcaatggttgatctgagctggtggctacataataaacacgaacatttgtgtcttcacagccagtggctatcatgtctttattgttttggctccaatcacaaccaaacactgcagctggatgtttatatttgtgtagcactttaccatcaattgttcgaataatacagaaaccatcactgctgcaggttgctattcttttagaatctttatgactccaggcaatgcagaatattccatttgttccatgctcattaaatcgttgtataattttgcccttttgaacattccaaataaaagcaccatttcgggaagttcccccagcaatacaatttaaaccacctggagcccaagaaagggaataaataacaccttcattacccggggatgtgtacactgctgttaatgtgtttatatcccagacttttatagtgccatcaaatgaagctgttgctaaaagattaggatcgtcaggtttgaatttgcagtcaaagatagtttccacatgtcccaagtctctaagaaaatcccacttcttagctcccatatcataaagtccaactccaccatccaagaaacaacacactgcatgaccaggaggaagagaaaatgcttgattctgtgttaaagttgggggtggaactgcttcgcttgttgaggatgtataatgatttttggttggagattggactgaaaacttttttcttggaggagaattaagtacatgtaagcagtgaaatcctgttttctttaatttaagattatcaataggtgttgttcttgaaacattccaaatgcgtaaaacacccacttgagaatctccagttataaacatcccaggagcactgggaacccaggctaagcactgtacagaagctgctgcactgggaagattaaatgttgttatgcaagaaagtgattcagaatctaccaggcgaattccataatgcaaattaaccactagaagataatcagtagatagtgggtcccattccaaggccgtaactggatcctcttcatctgtcccttcaagagattctggtctcaaaacatgtttctgatttttattacctggatgaaaaattgatagacttccatcaatatgaccaaacacaactttccccttttggtgtgtatgccatctgaacatacagatatcagacaagaagctatgagcatctttgtgtacaatcactccactatctggtcctgagatggtccaaatgaacagtgggcctctgtgggaaacaaatgccaccacatcctctgcattccagcaccaactaagagaagcagggatcccttttgtactgtcgagtttagcaatgactttttgttctgcaacattccaaatgatcactaaattatcagtactgccacttgcaaacagatcaggattatgtggacaccaagaaattgctgtgattgtttttttatgttcagacataattgcgtgaagtttgaattcattataacggtgatccaactgataaatatagatagccagggtcgcacaatatgcaaacctgtctccactggcagcacatacatccttgttccatggctgacatccagcagccagcaatcccacttgccttacctgggacatgtttgctctttgtagtccttcataccaatcatcttgctcaaaccaatttgaaatgtaagtcatccaagccatagaatgtttctactttaatcaaggcaattggaaactcggcatcagaatagtcagcacctaaagtaacaacaatgtgtttcaaccaaacaagatttaccaaaatctcccttgtgaaatgatgttcagtacaaaaggctagaactgcacaaatattt

SEQ ID NO: 10825 - RNA, 5714 nt, Homo sapiens
  source 1..5714: mol_type = other RNA
ctgaatagctgggactacaggtacacaccaccacacccagctaatttttgtatttttagtagagacagggtttcaccatgttggccaggatggtctccatctaccgacctcaagatctgcccatctcggcctcctgaagtgctgggattacaggcaattttttttttttaataaaatggaatttaagcctgtaatgtctttttaaggaatcaaaagtggtcatgtgataaatatgatacatagatacataatatatattttttccagttttaagaagttttgttaagaaggttttaaaaatattttaaatgcaacaagtttaaagataataaaagccacaagtattctagttatatgagattattctttagtcaaacaaaaccatctatattataaatcttgtgaaacaacttgagtatcaaagtacttccagtatgcattaatttaataagtttcaaagtcagaattctagtccaactgaaatatctgtagtcacattatcaggcttttcatagcttcacacttttaaacaacattttaaaagttaaatcaacataatatatccaaaaattcaaccaatatctatttacaaacatttacttaaaactaattttcatcaaatcaattgtggtttttgttggtttgttttttgagacagagtttcgctctttgttgcccaggctggagtgcagtggtgcgatcttggctcactggaacctctgcctcccaggttcaagggattctcctgcctcagcttcccaagtaactgggattacaggtgcccgccaccatgcctggctaatttttgtatttttagtggagacagggttttaccatgctggccaggctggtcatgaactcctgacctcaggtgatccacctgccttggcctgccaaagtgctgagattacaggtgtgagccaccgtgcccggccaaataaattgtgttttaaataaagttaacataaattgactagagtatactgtgtaaattattgtacacattaatcaaaactaatatccatgcatgctgaatctcttaaaatagtcactttatcacctaatgcaagttttcatatatatattcgactgcattttgtgatttttacccgccaatttttttcaagcctatataacttacacctttacaatgggacagttaaacttcagataaaaaaactggtaacattttcttttttttaaaagtattttgaatgtgtatccatttattaatatttactaaacttataactgaaaacttttattaaaacagctaacgttagtggtttactatgcattttataaaggagaacgtaagtgtttgttaagttgaagatcactgtgcacaccttacatttcaacatttcaagatattcaatcattcaaatatccattaagtacttactgtatgtctagcactattctaggtgttgcacaatttaatatgtttcaatatttcaaccatatgatattttggtatcttttatgctgtgtgaaacttttatatgctttttagattattcagtcctttataatttaaatgtttcctccttcccaaacgtagctattactgtttataaaggaggcacctatttttcctttaaattatatatatatatatattttgaagttaatgactaaaattcactgctatttcccacctctcccaacctgcaatccttctcccaacctctggcacttgagcaacaaagattaaggtaatgctaacccatgaaagtttttctttaaaaaaaaaaatcaagcatggacaaaaatcttctatcagaatggattgagtcgtattccagtccctaaaggtgagaatggattcacctttgcccacatcaaagcatcattcaaggagatagcagatttcccgtcttcaaggaaaaacacagggccctggatttttaatcccgtaagacaagaaatgtgaatatcagaatgacttggaagatttgatccagtcacataatctggtccaataattcctttcagtgactcttcttttagtctctttaataaagttgcataaatcattctttgtgaatcagaagggggtgtatacggagagtcttctaatgatctgttggtggactgtgtgcaagctctccatgcatccaattcctcagaaagatattcaatttttaaaggtactgacacctcccgacgttttaatagctgacttgtgtactcataaagtgctggaacaatgctttggtactgtcttctgatagccagtaatgcaccaatgtaaccacataatatcagcaactcatttcgagcttcagtacacgtatgcaagagtaatttttcagtacgaatatagctcagtaggtcaagaacagggtatatggtatccaaagtccagtctgagctactgatgtattctttaacaaagctaataccaataggaagggctttttcaggttcttgacttaacaagtaatattttacagtttcaaatatattgtcatctgcacgggctgtctcagctaactgcatacattcttccactgtgggtagcttacacttatcatgaaggtcatttatctcttcagtacatcctgggtagaaagcacagagttttattaaatgtagttcattatcaggaatcatcagaagaagatcagctgccaaattccatactgaaatcatcatgcactttctcgccagtaattctaaggcatagtgggttgctggtgctgcagactctcctagtactgtgcccacacagactgccaactccagttcatttccgcgaatcaggtatgccatagcaagctcaatattatctatggcaagatggcaacatgcggctagtactgctcgaccatcttgaaaataccattctgccagttctttactgactttgtgcaggagttcattaaagtcttccttgtagatatcatcagaatatgaagctcctttaggcacggaaacatgtaagggctgcatatttccttcacaagcagcctgtgcaacaagcagagcttctttaagctgacctcttgacatgaaaaaatggactagctttttcacatcaccaatggctatgcagtatggaatgacatcatccttatcttcctggattaattggtcagctctcctctgcattaacttcttccagtatttcacagagactcctggtgcaattgacagggctttgtcccactctccaagttcaaccataagttcacagtatctctgaatttgtcctaatctcaagtggatttcagcagcttccttcagtctttcctctttagcaggtacaccaataccaccaccaaatttagacatcttgactgttgttagttcttgagcttcagatgttctaaatttaatcagatgtttcaagtgcattattcctttgcagtagttctgaggaagtaagctatcatcctgtccttttatcacagcaaccaagttccataaattgtcactgccacctggaggagataaacattctgagaaccatcttagttttttcacttgagaattagcagttagtttttctatttcctgtctaatatctcttgacactttaccacacagtagaggaggagtgcctggttctatagcataatcagtgttcccaataatttcttcccaagatctgtctgccagaatatttatttgtacaggagtgactaaggctgttaatgaccagagtctcactgtagagtcacgggagcaagaggccatagtgaaggggcgactgggatggcaggttaaaccatatacatctgcaccgtgatcatacacagtatccacacaagttccttctcgagtgtcccatacttttatagtatagtcccagctgccagatatgagcagatatggaatctcagtattccacattaatcctctcacaggtgcagtgtgtccattaagaatattgatgcaagcatcctgagtataatcccagattcgaacggtattattgttttggctccaatcacaaccaaacactgcagctggatgtttatatttgtgtagcactttaccatcaattgttcgaataatacagaaaccatcactgctgcaggttgctattcttttagaatctttatgactccaggcaatgcagaatattccatttgttccatgctcattaaatcgttgtataattttgcccttttgaacattccaaataaaagcaccatttcgggaagttcccccagcaatacaatttaaaccacctggagcccaagaaagggaataaataacaccttcattacccggggatgtgtacactgctgttaatgtgtttatatcccagacttttatagtgccatcaaatgaagctgttgctaaaagattaggatcgtcaggtttgaatttgcagtcaaagatagtttccacatgtcccaagtctctaagaaaatcccacttcttagctcccatatcataaagtccaactccaccatccaagaaacaacacactgcatgaccaggaggaagagaaaatgcttgattctgtgttaaagttgggggtggaactgcttcgcttgttgaggatgtataatgatttttggttggagattggactgaaaacttttttcttggaggagaattaagtacatgtaagcagtgaaatcctgttttctttaatttaagattatcaataggtgttgttcttgaaacattccaaatgcgtaaaacacccacttgagaatctccagttataaacatcccaggagcactgggaacccaggctaagcactgtacagaagctgctgcactgggaagattaaatgttgttatgcaagaaagtgattcagaatctaccaggcgaattccataatgcaaattaaccactagaagataatcagtagatagtgggtcccattccaaggccgtaactggatcctcttcatctgtcccttcaagagattctggtctcaaaacatgtttctgatttttattacctggatgaaaaattgatagacttccatcaatatgaccaaacacaactttccccttttggtgtgtatgccatctgaacatacagatatcagacaagaagctatgagcatctttgtgtacaatcactccactatctggtcctgagatggtccaaatgaacagtgggcctctgtgggaaacaaatgccaccacatcctctgcattccagcaccaactaagagaagcagggatcccttttgtactgtcgagtttagcaatgactttttgttctgcaacattccaaatgatcactaaattatcagtactgccacttgcaaacagatcaggattatgtggacaccaagaaattgctgtgattgtttttttatgttcagacataattgcgtgaagtttgaattcattataacggtgatccaactgataaatatagatagccagggtcgcacaatatgcaaacctgtctccactggcagcacatacatccttgttccatggctgacatccagcagccagcaatcccacttgccttacctgggacatgtttgcctggaggaggaggcggctgcagcggcggacagcggaaggtgctgaagccggcgggcgcagctgcgaggcgagcaccaccaacgcgcggaccctccccgccctccccgcctgctcgctcagggcgcccgggggcggggcggccgggcccgcgggctccgaggggcgggaagcgtgctccgcaagccccagcgcggagccacgatggaaggcgccgcgagcccgatctccagggtctgccc

SEQ ID NO: 10826 - RNA, 5696 nt, Homo sapiens
  source 1..5696: mol_type = other RNA
ctgaatagctgggactacaggtacacaccaccacacccagctaatttttgtatttttagtagagacagggtttcaccatgttggccaggatggtctccatctaccgacctcaagatctgcccatctcggcctcctgaagtgctgggattacaggcaattttttttttttaataaaatggaatttaagcctgtaatgtctttttaaggaatcaaaagtggtcatgtgataaatatgatacatagatacataatatatattttttccagttttaagaagttttgttaagaaggttttaaaaatattttaaatgcaacaagtttaaagataataaaagccacaagtattctagttatatgagattattctttagtcaaacaaaaccatctatattataaatcttgtgaaacaacttgagtatcaaagtacttccagtatgcattaatttaataagtttcaaagtcagaattctagtccaactgaaatatctgtagtcacattatcaggcttttcatagcttcacacttttaaacaacattttaaaagttaaatcaacataatatatccaaaaattcaaccaatatctatttacaaacatttacttaaaactaattttcatcaaatcaattgtggtttttgttggtttgttttttgagacagagtttcgctctttgttgcccaggctggagtgcagtggtgcgatcttggctcactggaacctctgcctcccaggttcaagggattctcctgcctcagcttcccaagtaactgggattacaggtgcccgccaccatgcctggctaatttttgtatttttagtggagacagggttttaccatgctggccaggctggtcatgaactcctgacctcaggtgatccacctgccttggcctgccaaagtgctgagattacaggtgtgagccaccgtgcccggccaaataaattgtgttttaaataaagttaacataaattgactagagtatactgtgtaaattattgtacacattaatcaaaactaatatccatgcatgctgaatctcttaaaatagtcactttatcacctaatgcaagttttcatatatatattcgactgcattttgtgatttttacccgccaatttttttcaagcctatataacttacacctttacaatgggacagttaaacttcagataaaaaaactggtaacattttcttttttttaaaagtattttgaatgtgtatccatttattaatatttactaaacttataactgaaaacttttattaaaacagctaacgttagtggtttactatgcattttataaaggagaacgtaagtgtttgttaagttgaagatcactgtgcacaccttacatttcaacatttcaagatattcaatcattcaaatatccattaagtacttactgtatgtctagcactattctaggtgttgcacaatttaatatgtttcaatatttcaaccatatgatattttggtatcttttatgctgtgtgaaacttttatatgctttttagattattcagtcctttataatttaaatgtttcctccttcccaaacgtagctattactgtttataaaggaggcacctatttttcctttaaattatatatatatatatattttgaagttaatgactaaaattcactgctatttcccacctctcccaacctgcaatccttctcccaacctctggcacttgagcaacaaagattaaggtaatgctaacccatgaaagtttttctttaaaaaaaaaaatcaagcatggacaaaaatcttctatcagaatggattgagtcgtattccagtccctaaaggtgagaatggattcacctttgcccacatcaaagcatcattcaaggagatagcagatttcccgtcttcaaggaaaaacacagggccctggatttttaatcccgtaagacaagaaatgtgaatatcagaatgacttggaagatttgatccagtcacataatctggtccaataattcctttcagtgactcttcttttagtctctttaataaagttgcataaatcattctttgtgaatcagaagggggtgtatacggagagtcttctaatgatctgttggtggactgtgtgcaagctctccatgcatccaattcctcagaaagatattcaatttttaaaggtactgacacctcccgacgttttaatagctgacttgtgtactcataaagtgctggaacaatgctttggtactgtcttctgatagccagtaatgcaccaatgtaaccacataatatcagcaactcatttcgagcttcagtacacgtatgcaagagtaatttttcagtacgaatatagctcagtaggtcaagaacagggtatatggtatccaaagtccagtctgagctactgatgtattctttaacaaagctaataccaataggaagggctttttcaggttcttgacttaacaagtaatattttacagtttcaaatatattgtcatctgcacgggctgtctcagctaactgcatacattcttccactgtgggtagcttacacttatcatgaaggtcatttatctcttcagtacatcctgggtagaaagcacagagttttattaaatgtagttcattatcaggaatcatcagaagaagatcagctgccaaattccatactgaaatcatcatgcactttctcgccagtaattctaaggcatagtgggttgctggtgctgcagactctcctagtactgtgcccacacagactgccaactccagttcatttccgcgaatcaggtatgccatagcaagctcaatattatctatggcaagatggcaacatgcggctagtactgctcgaccatcttgaaaataccattctgccagttctttactgactttgtgcaggagttcattaaagtcttccttgtagatatcatcagaatatgaagctcctttaggcacggaaacatgtaagggctgcatatttccttcacaagcagcctgtgcaacaagcagagcttctttaagctgacctcttgacatgaaaaaatggactagctttttcacatcaccaatggctatgcagtatggaatgacatcatccttatcttcctggattaattggtcagctctcctctgcattaacttcttccagtatttcacagagactcctggtgcaattgacagggctttgtcccactctccaagttcaaccataagttcacagtatctctgaatttgtcctaatctcaagtggatttcagcagcttccttcagtctttcctctttagcaggtacaccaataccaccaccaaatttagacatcttgactgttgttagttcttgagcttcagatgttctaaatttaatcagatgtttcaagtgcattattcctttgcagtagttctgaggaagtaagctatcatcctgtccttttatcacagcaaccaagttccataaattgtcactgccacctggaggagataaacattctgagaaccatcttagttttttcacttgagaattagcagttagtttttctatttcctgtctaatatctcttgacactttaccacacagtagaggaggagtgcctggttctatagcataatcagtgttcccaataatttcttcccaagatctgtctgccagaatatttatttgtacaggagtgactaaggctgttaatgaccagagtctcactgtagagtcacgggagcaagaggccatagtgaaggggcgactgggatggcaggttaaaccatatacatctgcaccgtgatcatacacagtatccacacaagttccttctcgagtgtcccatacttttatagtatagtcccagctgccagatatgagcagatatggaatctcagtattccacattaatcctctcacaggtgcagtgtgtccattaagaatattgatgcaagcatcctgagtataatcccagattcgaacggtattattgttttggctccaatcacaaccaaacactgcagctggatgtttatatttgtgtagcactttaccatcaattgttcgaataatacagaaaccatcactgctgcaggttgctattcttttagaatctttatgactccaggcaatgcagaatattccatttgttccatgctcattaaatcgttgtataattttgcccttttgaacattccaaataaaagcaccatttcgggaagttcccccagcaatacaatttaaaccacctggagcccaagaaagggaataaataacaccttcattacccggggatgtgtacactgctgttaatgtgtttatatcccagacttttatagtgccatcaaatgaagctgttgctaaaagattaggatcgtcaggtttgaatttgcagtcaaagatagtttccacatgtcccaagtctctaagaaaatcccacttcttagctcccatatcataaagtccaactccaccatccaagaaacaacacactgcatgaccaggaggaagagaaaatgcttgattctgtgttaaagttgggggtggaactgcttcgcttgttgaggatgtataatgatttttggttggagattggactgaaaacttttttcttggaggagaattaagtacatgtaagcagtgaaatcctgttttctttaatttaagattatcaataggtgttgttcttgaaacattccaaatgcgtaaaacacccacttgagaatctccagttataaacatcccaggagcactgggaacccaggctaagcactgtacagaagctgctgcactgggaagattaaatgttgttatgcaagaaagtgattcagaatctaccaggcgaattccataatgcaaattaaccactagaagataatcagtagatagtgggtcccattccaaggccgtaactggatcctcttcatctgtcccttcaagagattctggtctcaaaacatgtttctgatttttattacctggatgaaaaattgatagacttccatcaatatgaccaaacacaactttccccttttggtgtgtatgccatctgaacatacagatatcagacaagaagctatgagcatctttgtgtacaatcactccactatctggtcctgagatggtccaaatgaacagtgggcctctgtgggaaacaaatgccaccacatcctctgcattccagcaccaactaagagaagcagggatcccttttgtactgtcgagtttagcaatgactttttgttctgcaacattccaaatgatcactaaattatcagtactgccacttgcaaacagatcaggattatgtggacaccaagaaattgctgtgattgtttttttatgttcagacataattgcgtgaagtttgaattcattataacggtgatccaactgataaatatagatagccagggtcgcacaatatgcaaacctgtctccactggcagcacatacatccttgttccatggctgacatccagcagccagcaatcccacttgccttacctgggacatgtttgctctttgtagtccttcataccaatcatcttgctcaaaccaatttgaaatgtaagtcatccaagccatagaatgtttctactttaatcaaggcaattggaaactcggcatcagaatagtcagcacctaaagtaacaacaatgtgtttcaaccaaacaagatttaccaaaatctcccttgtgaaatgatgttcagtacaaaaggctagaactgcacaaatattt

SEQ ID NO: 10827 - RNA, 5680 nt, Homo sapiens
  source 1..5680: mol_type = other RNA
ctgaatagctgggactacaggtacacaccaccacacccagctaatttttgtatttttagtagagacagggtttcaccatgttggccaggatggtctccatctaccgacctcaagatctgcccatctcggcctcctgaagtgctgggattacaggcaattttttttttttaataaaatggaatttaagcctgtaatgtctttttaaggaatcaaaagtggtcatgtgataaatatgatacatagatacataatatatattttttccagttttaagaagttttgttaagaaggttttaaaaatattttaaatgcaacaagtttaaagataataaaagccacaagtattctagttatatgagattattctttagtcaaacaaaaccatctatattataaatcttgtgaaacaacttgagtatcaaagtacttccagtatgcattaatttaataagtttcaaagtcagaattctagtccaactgaaatatctgtagtcacattatcaggcttttcatagcttcacacttttaaacaacattttaaaagttaaatcaacataatatatccaaaaattcaaccaatatctatttacaaacatttacttaaaactaattttcatcaaatcaattgtggtttttgttggtttgttttttgagacagagtttcgctctttgttgcccaggctggagtgcagtggtgcgatcttggctcactggaacctctgcctcccaggttcaagggattctcctgcctcagcttcccaagtaactgggattacaggtgcccgccaccatgcctggctaatttttgtatttttagtggagacagggttttaccatgctggccaggctggtcatgaactcctgacctcaggtgatccacctgccttggcctgccaaagtgctgagattacaggtgtgagccaccgtgcccggccaaataaattgtgttttaaataaagttaacataaattgactagagtatactgtgtaaattattgtacacattaatcaaaactaatatccatgcatgctgaatctcttaaaatagtcactttatcacctaatgcaagttttcatatatatattcgactgcattttgtgatttttacccgccaatttttttcaagcctatataacttacacctttacaatgggacagttaaacttcagataaaaaaactggtaacattttcttttttttaaaagtattttgaatgtgtatccatttattaatatttactaaacttataactgaaaacttttattaaaacagctaacgttagtggtttactatgcattttataaaggagaacgtaagtgtttgttaagttgaagatcactgtgcacaccttacatttcaacatttcaagatattcaatcattcaaatatccattaagtacttactgtatgtctagcactattctaggtgttgcacaatttaatatgtttcaatatttcaaccatatgatattttggtatcttttatgctgtgtgaaacttttatatgctttttagattattcagtcctttataatttaaatgtttcctccttcccaaacgtagctattactgtttataaaggaggcacctatttttcctttaaattatatatatatatatattttgaagttaatgactaaaattcactgctatttcccacctctcccaacctgcaatccttctcccaacctctggcacttgagcaacaaagattaaggtaatgctaacccatgaaagtttttctttaaaaaaaaaaatcaagcatggacaaaaatcttctatcagaatggattgagtcgtattccagtccctaaaggtgagaatggattcacctttgcccacatcaaagcatcattcaaggagatagcagatttcccgtcttcaaggaaaaacacagggccctggatttttaatcccgtaagacaagaaatgtgaatatcagaatgacttggaagatttgatccagtcacataatctggtccaataattcctttcagtgactcttcttttagtctctttaataaagttgcataaatcattctttgtgaatcagaagggggtgtatacggagagtcttctaatgatctgttggtggactgtgtgcaagctctccatgcatccaattcctcagaaagatattcaatttttaaaggtactgacacctcccgacgttttaatagctgacttgtgtactcataaagtgctggaacaatgctttggtactgtcttctgatagccagtaatgcaccaatgtaaccacataatatcagcaactcatttcgagcttcagtacacgtatgcaagagtaatttttcagtacgaatatagctcagtaggtcaagaacagggtatatggtatccaaagtccagtctgagctactgatgtattctttaacaaagctaataccaataggaagggctttttcaggttcttgacttaacaagtaatattttacagtttcaaatatattgtcatctgcacgggctgtctcagctaactgcatacattcttccactgtgggtagcttacacttatcatgaaggtcatttatctcttcagtacatcctgggtagaaagcacagagttttattaaatgtagttcattatcaggaatcatcagaagaagatcagctgccaaattccatactgaaatcatcatgcactttctcgccagtaattctaaggcatagtgggttgctggtgctgcagactctcctagtactgtgcccacacagactgccaactccagttcatttccgcgaatcaggtatgccatagcaagctcaatattatctatggcaagatggcaacatgcggctagtactgctcgaccatcttgaaaataccattctgccagttctttactgactttgtgcaggagttcattaaagtcttccttgtagatatcatcagaatatgaagctcctttaggcacggaaacatgtaagggctgcatatttccttcacaagcagcctgtgcaacaagcagagcttctttaagctgacctcttgacatgaaaaaatggactagctttttcacatcaccaatggctatgcagtatggaatgacatcatccttatcttcctggattaattggtcagctctcctctgcattaacttcttccagtatttcacagagactcctggtgcaattgacagggctttgtcccactctccaagttcaaccataagttcacagtatctctgaatttgtcctaatctcaagtggatttcagcagcttccttcagtctttcctctttagcaggtacaccaataccaccaccaaatttagacatcttgactgttgttagttcttgagcttcagatgttctaaatttaatcagatgtttcaagtgcattattcctttgcagtagttctgaggaagtaagctatcatcctgtccttttatcacagcaaccaagttccataaattgtcactgccacctggaggagataaacattctgagaaccatcttagttttttcacttgagaattagcagttagtttttctatttcctgtctaatatctcttgacactttaccacacagtagaggaggagtgcctggttctatagcataatcagtgttcccaataatttcttcccaagatctgtctgccagaatatttatttgtacaggagtgactaaggctgttaatgaccagagtctcactgtagagtcacgggagcaagaggccatagtgaaggggcgactgggatggcaggttaaaccatatacatctgcaccgtgatcatacacagtatccacacaagttccttctcgagtgtcccatacttttatagtatagtcccagctgccagatatgagcagatatggaatctcagtattccacattaatcctctcacaggtgcagtgtgtccattaagaatattgatgcaagcatcctgagtataatcccagattcgaacggtattattgttttggctccaatcacaaccaaacactgcagctggatgtttatatttgtgtagcactttaccatcaattgttcgaataatacagaaaccatcactgctgcaggttgctattcttttagaatctttatgactccaggcaatgcagaatattccatttgttccatgctcattaaatcgttgtataattttgcccttttgaacattccaaataaaagcaccatttcgggaagttcccccagcaatacaatttaaaccacctggagcccaagaaagggaataaataacaccttcattacccggggatgtgtacactgctgttaatgtgtttatatcccagacttttatagtgccatcaaatgaagctgttgctaaaagattaggatcgtcaggtttgaatttgcagtcaaagatagtttccacatgtcccaagtctctaagaaaatcccacttcttagctcccatatcataaagtccaactccaccatccaagaaacaacacactgcatgaccaggaggaagagaaaatgcttgattctgtgttaaagttgggggtggaactgcttcgcttgttgaggatgtataatgatttttggttggagattggactgaaaacttttttcttggaggagaattaagtacatgtaagcagtgaaatcctgttttctttaatttaagattatcaataggtgttgttcttgaaacattccaaatgcgtaaaacacccacttgagaatctccagttataaacatcccaggagcactgggaacccaggctaagcactgtacagaagctgctgcactgggaagattaaatgttgttatgcaagaaagtgattcagaatctaccaggcgaattccataatgcaaattaaccactagaagataatcagtagatagtgggtcccattccaaggccgtaactggatcctcttcatctgtcccttcaagagattctggtctcaaaacatgtttctgatttttattacctggatgaaaaattgatagacttccatcaatatgaccaaacacaactttccccttttggtgtgtatgccatctgaacatacagatatcagacaagaagctatgagcatctttgtgtacaatcactccactatctggtcctgagatggtccaaatgaacagtgggcctctgtgggaaacaaatgccaccacatcctctgcattccagcaccaactaagagaagcagggatcccttttgtactgtcgagtttagcaatgactttttgttctgcaacattccaaatgatcactaaattatcagtactgccacttgcaaacagatcaggattatgtggacaccaagaaattgctgtgattgtttttttatgttcagacataattgcgtgaagtttgaattcattataacggtgatccaactgataaatatagatagccagggtcgcacaatatgcaaacctgtctccactggcagcacatacatccttgttccatggctgacatccagcagccagcaatcccacttgccttacctgggacatgtttgctctttgtagtccttcataccaatcatcttgctcaaaccaatttgaaatgtaagtcatccaagccatagaatgtttctactttaatcaaggcaattggaaactcggcatcagaatagtcagcacctggaggaggaggcggctgcagcggcggacagcggaaggtgctgaagccggcgggcgcagctgcgaggcgagcaccaccaac

SEQ ID NO: 10828 - RNA, 5972 nt, Homo sapiens
  source 1..5972: mol_type = other RNA
ctgaatagctgggactacaggtacacaccaccacacccagctaatttttgtatttttagtagagacagggtttcaccatgttggccaggatggtctccatctaccgacctcaagatctgcccatctcggcctcctgaagtgctgggattacaggcaattttttttttttaataaaatggaatttaagcctgtaatgtctttttaaggaatcaaaagtggtcatgtgataaatatgatacatagatacataatatatattttttccagttttaagaagttttgttaagaaggttttaaaaatattttaaatgcaacaagtttaaagataataaaagccacaagtattctagttatatgagattattctttagtcaaacaaaaccatctatattataaatcttgtgaaacaacttgagtatcaaagtacttccagtatgcattaatttaataagtttcaaagtcagaattctagtccaactgaaatatctgtagtcacattatcaggcttttcatagcttcacacttttaaacaacattttaaaagttaaatcaacataatatatccaaaaattcaaccaatatctatttacaaacatttacttaaaactaattttcatcaaatcaattgtggtttttgttggtttgttttttgagacagagtttcgctctttgttgcccaggctggagtgcagtggtgcgatcttggctcactggaacctctgcctcccaggttcaagggattctcctgcctcagcttcccaagtaactgggattacaggtgcccgccaccatgcctggctaatttttgtatttttagtggagacagggttttaccatgctggccaggctggtcatgaactcctgacctcaggtgatccacctgccttggcctgccaaagtgctgagattacaggtgtgagccaccgtgcccggccaaataaattgtgttttaaataaagttaacataaattgactagagtatactgtgtaaattattgtacacattaatcaaaactaatatccatgcatgctgaatctcttaaaatagtcactttatcacctaatgcaagttttcatatatatattcgactgcattttgtgatttttacccgccaatttttttcaagcctatataacttacacctttacaatgggacagttaaacttcagataaaaaaactggtaacattttcttttttttaaaagtattttgaatgtgtatccatttattaatatttactaaacttataactgaaaacttttattaaaacagctaacgttagtggtttactatgcattttataaaggagaacgtaagtgtttgttaagttgaagatcactgtgcacaccttacatttcaacatttcaagatattcaatcattcaaatatccattaagtacttactgtatgtctagcactattctaggtgttgcacaatttaatatgtttcaatatttcaaccatatgatattttggtatcttttatgctgtgtgaaacttttatatgctttttagattattcagtcctttataatttaaatgtttcctccttcccaaacgtagctattactgtttataaaggaggcacctatttttcctttaaattatatatatatatatattttgaagttaatgactaaaattcactgctatttcccacctctcccaacctgcaatccttctcccaacctctggcacttgagcaacaaagattaaggtaatgctaacccatgaaagtttttctttaaaaaaaaaaatcaagcatggacaaaaatcttctatcagaatggattgagtcgtattccagtccctaaaggtgagaatggattcacctttgcccacatcaaagcatcattcaaggagatagcagatttcccgtcttcaaggaaaaacacagggccctggatttttaatcccgtaagacaagaaatgtgaatatcagaatgacttggaagatttgatccagtcacataatctggtccaataattcctttcagtgactcttcttttagtctctttaataaagttgcataaatcattctttgtgaatcagaagggggtgtatacggagagtcttctaatgatctgttggtggactgtgtgcaagctctccatgcatccaattcctcagaaagatattcaatttttaaaggtactgacacctcccgacgttttaatagctgacttgtgtactcataaagtgctggaacaatgctttggtactgtcttctgatagccagtaatgcaccaatgtaaccacataatatcagcaactcatttcgagcttcagtacacgtatgcaagagtaatttttcagtacgaatatagctcagtaggtcaagaacagggtatatggtatccaaagtccagtctgagctactgatgtattctttaacaaagctaataccaataggaagggctttttcaggttcttgacttaacaagtaatattttacagtttcaaatatattgtcatctgcacgggctgtctcagctaactgcatacattcttccactgtgggtagcttacacttatcatgaaggtcatttatctcttcagtacatcctgggtagaaagcacagagttttattaaatgtagttcattatcaggaatcatcagaagaagatcagctgccaaattcctgtatccaacacatggaaagcatactgaaatcatcatgcactttctcgccagtaattctaaggcatagtgggttgctggtgctgcagactctcctagtactgtgcccacacagactgccaactccagttcatttccgcgaatcaggtatgccatagcaagctcaatattatctatggcaagatggcaacatgcggctagtactgctcgaccatcttgaaaataccattctgccagttctttactgactttgtgcaggagttcattaaagtcttccttgtagatatcatcagaatatgaagctcctttaggcacggaaacatgtaagggctgcatatttccttcacaagcagcctgtgcaacaagcagagcttctttaagctgacctcttgacatgaaaaaatggactagctttttcacatcaccaatggctatgcagtatggaatgacatcatccttatcttcctggattaattggtcagctctcctctgcattaacttcttccagtatttcacagagactcctggtgcaattgacagggctttgtcccactctccaagttcaaccataagttcacagtatctctgaatttgtcctaatctcaagtggatttcagcagcttccttcagtctttcctctttagcaggtacaccaataccaccaccaaatttagacatcttgactgttgttagttcttgagcttcagatgttctaaatttaatcagatgtttcaagtgcattattcctttgcagtagttctgaggaagtaagctatcatcctgtccttttatcacagcaaccaagttccataaattgtcactgccacctggaggagataaacattctgagaaccatcttagttttttcacttgagaattagcagttagtttttctatttcctgtctaatatctcttgacactttaccacacagtagaggaggagtgcctggttctatagcataatcagtgttcccaataatttcttcccaagatctgtctgccagaatatttatttgtacaggagtgactaaggctgttaatgaccagagtctcactgtagagtcacgggagcaagaggccatagtgaaggggcgactgggatggcaggttaaaccatatacatctgcaccgtgatcatacacagtatccacacaagttccttctcgagtgtcccatacttttatagtatagtcccagctgccagatatgagcagatatggaatctcagtattccacattaatcctctcacaggtgcagtgtgtccattaagaatattgatgcaagcatcctgagtataatcccagattcgaacggtaccatcatcagaaccactgcaaagaattccctctctcagaggagaccatttaacatgaaacacttttgctgtatgcccactaaatactttcaatggttgatctgagctggtggctacataataaacacgaacatttgtgtcttcacagccagtggctatcatgtctttattgttttggctccaatcacaaccaaacactgcagctggatgtttatatttgtgtagcactttaccatcaattgttcgaataatacagaaaccatcactgctgcaggttgctattcttttagaatctttatgactccaggcaatgcagaatattccatttgttccatgctcattaaatcgttgtataattttgcccttttgaacattccaaataaaagcaccatttcgggaagttcccccagcaatacaatttaaaccacctggagcccaagaaagggaataaataacaccttcattacccggggatgtgtacactgctgttaatgtgtttatatcccagacttttatagtgccatcaaatgaagctgttgctaaaagattaggatcgtcaggtttgaatttgcagtcaaagatagtttccacatgtcccaagtctctaagaaaatcccacttcttagctcccatatcataaagtccaactccaccatccaagaaacaacacactgcatgaccaggaggaagagaaaatgcttgattctgtgttaaagttgggggtggaactgcttcgcttgttgaggatgtataatgatttttggttggagattggactgaaaacttttttcttggaggagaattaagtacatgtaagcagtgaaatcctgttttctttaatttaagattatcaataggtgttgttcttgaaacattccaaatgcgtaaaacacccacttgagaatagttctgcatggctgaggaggcctcaggaaacttacaatcatggtggaaggcaaagtagaagcaggcaccttctccagttataaacatcccaggagcactgggaacccaggctaagcactgtacagaagctgctgcactgggaagattaaatgttgttatgcaagaaagtgattcagaatctaccaggcgaattccataatgcaaattaaccactagaagataatcagtagatagtgggtcccattccaaggccgtaactggatcctcttcatctgtcccttcaagagattctggtctcaaaacatgtttctgatttttattacctggatgaaaaattgatagacttccatcaatatgaccaaacacaactttccccttttggtgtgtatgccatctgaacatacagatatcagacaagaagctatgagcatctttgtgtacaatcactccactatctggtcctgagatggtccaaatgaacagtgggcctctgtgggaaacaaatgccaccacatcctctgcattccagcaccaactaagagaagcagggatcccttttgtactgtcgagtttagcaatgactttttgttctgcaacattccaaatgatcactaaattatcagtactgccacttgcaaacagatcaggattatgtggacaccaagaaattgctgtgattgtttttttatgttcagacataattgcgtgaagtttgaattcattataacggtgatccaactgataaatatagatagccagggtcgcacaatatgcaaacctgtctccactggcagcacatacatccttgttccatggctgacatccagcagccagcaatcccacttgccttacctgggacatgtttgcctggaggaggaggcggctgcagcggcggacagcggaaggtgctgaagccggcgggcgcagctgcgaggcgagcaccaccaacgcgcggaccctccccgccctccccgcctgctcgctcagggcgcccgggggcggggcggccgggcccgcgggctccgaggggcgggaagcgtgctccgcaagccccagcgcggagccacgatggaaggcgccgcgagcccgatctccagggtctgccc

SEQ ID NO: 10829 - RNA, 5955 nt, Homo sapiens
  source 1..5955: mol_type = other RNA
ctgaatagctgggactacaggtacacaccaccacacccagctaatttttgtatttttagtagagacagggtttcaccatgttggccaggatggtctccatctaccgacctcaagatctgcccatctcggcctcctgaagtgctgggattacaggcaattttttttttttaataaaatggaatttaagcctgtaatgtctttttaaggaatcaaaagtggtcatgtgataaatatgatacatagatacataatatatattttttccagttttaagaagttttgttaagaaggttttaaaaatattttaaatgcaacaagtttaaagataataaaagccacaagtattctagttatatgagattattctttagtcaaacaaaaccatctatattataaatcttgtgaaacaacttgagtatcaaagtacttccagtatgcattaatttaataagtttcaaagtcagaattctagtccaactgaaatatctgtagtcacattatcaggcttttcatagcttcacacttttaaacaacattttaaaagttaaatcaacataatatatccaaaaattcaaccaatatctatttacaaacatttacttaaaactaattttcatcaaatcaattgtggtttttgttggtttgttttttgagacagagtttcgctctttgttgcccaggctggagtgcagtggtgcgatcttggctcactggaacctctgcctcccaggttcaagggattctcctgcctcagcttcccaagtaactgggattacaggtgcccgccaccatgcctggctaatttttgtatttttagtggagacagggttttaccatgctggccaggctggtcatgaactcctgacctcaggtgatccacctgccttggcctgccaaagtgctgagattacaggtgtgagccaccgtgcccggccaaataaattgtgttttaaataaagttaacataaattgactagagtatactgtgtaaattattgtacacattaatcaaaactaatatccatgcatgctgaatctcttaaaatagtcactttatcacctaatgcaagttttcatatatatattcgactgcattttgtgatttttacccgccaatttttttcaagcctatataacttacacctttacaatgggacagttaaacttcagataaaaaaactggtaacattttcttttttttaaaagtattttgaatgtgtatccatttattaatatttactaaacttataactgaaaacttttattaaaacagctaacgttagtggtttactatgcattttataaaggagaacgtaagtgtttgttaagttgaagatcactgtgcacaccttacatttcaacatttcaagatattcaatcattcaaatatccattaagtacttactgtatgtctagcactattctaggtgttgcacaatttaatatgtttcaatatttcaaccatatgatattttggtatcttttatgctgtgtgaaacttttatatgctttttagattattcagtcctttataatttaaatgtttcctccttcccaaacgtagctattactgtttataaaggaggcacctatttttcctttaaattatatatatatatatattttgaagttaatgactaaaattcactgctatttcccacctctcccaacctgcaatccttctcccaacctctggcacttgagcaacaaagattaaggtaatgctaacccatgaaagtttttctttaaaaaaaaaaatcaagcatggacaaaaatcttctatcagaatggattgagtcgtattccagtccctaaaggtgagaatggattcacctttgcccacatcaaagcatcattcaaggagatagcagatttcccgtcttcaaggaaaaacacagggccctggatttttaatcccgtaagacaagaaatgtgaatatcagaatgacttggaagatttgatccagtcacataatctggtccaataattcctttcagtgactcttcttttagtctctttaataaagttgcataaatcattctttgtgaatcagaagggggtgtatacggagagtcttctaatgatctgttggtggactgtgtgcaagctctccatgcatccaattcctcagaaagatattcaatttttaaaggtactgacacctcccgacgttttaatagctgacttgtgtactcataaagtgctggaacaatgctttggtactgtcttctgatagccagtaatgcaccaatgtaaccacataatatcagcaactcatttcgagcttcagtacacgtatgcaagagtaatttttcagtacgaatatagctcagtaggtcaagaacagggtatatggtatccaaagtccagtctgagctactgatgtattctttaacaaagctaataccaataggaagggctttttcaggttcttgacttaacaagtaatattttacagtttcaaatatattgtcatctgcacgggctgtctcagctaactgcatacattcttccactgtgggtagcttacacttatcatgaaggtcatttatctcttcagtacatcctgggtagaaagcacagagttttattaaatgtagttcattatcaggaatcatcagaagaagatcagctgccaaattcctgtatccaacacatggaaagcatactgaaatcatcatgcactttctcgccagtaattctaaggcatagtgggttgctggtgctgcagactctcctagtactgtgcccacacagactgccaactccagttcatttccgcgaatcaggtatgccatagcaagctcaatattatctatggcaagatggcaacatgcggctagtactgctcgaccatcttgaaaataccattctgccagttctttactgactttgtgcaggagttcattaaagtcttccttgtagatatcatcagaatatgaagctcctttaggcacggaaacatgtaagggctgcatatttccttcacaagcagcctgtgcaacaagcagagcttctttaagctgacctcttgacatgaaaaaatggactagctttttcacatcaccaatggctatgcagtatggaatgacatcatccttatcttcctggattaattggtcagctctcctctgcattaacttcttccagtatttcacagagactcctggtgcaattgacagggctttgtcccactctccaagttcaaccataagttcacagtatctctgaatttgtcctaatctcaagtggatttcagcagcttccttcagtctttcctctttagcaggtacaccaataccaccaccaaatttagacatcttgactgttgttagttcttgagcttcagatgttctaaatttaatcagatgtttcaagtgcattattcctttgcagtagttctgaggaagtaagctatcatcctgtccttttatcacagcaaccaagttccataaattgtcactgccacctggaggagataaacattctgagaaccatcttagttttttcacttgagaattagcagttagtttttctatttcctgtctaatatctcttgacactttaccacacagtagaggaggagtgcctggttctatagcataatcagtgttcccaataatttcttcccaagatctgtctgccagaatatttatttgtacaggagtgactaaggctgttaatgaccagagtctcactgtagagtcacgggagcaagaggccatagtgaaggggcgactgggatggcaggttaaaccatatacatctgcaccgtgatcatacacagtatccacacaagttccttctcgagtgtcccatacttttatagtatagtcccagctgccagatatgagcagatatggaatctcagtattccacattaatcctctcacaggtgcagtgtgtccattaagaatattgatgcaagcatcctgagtataatcccagattcgaacggtaccatcatcagaaccactgcaaagaattccctctctcagaggagaccatttaacatgaaacacttttgctgtatgcccactaaatactttcaatggttgatctgagctggtggctacataataaacacgaacatttgtgtcttcacagccagtggctatcatgtctttattgttttggctccaatcacaaccaaacactgcagctggatgtttatatttgtgtagcactttaccatcaattgttcgaataatacagaaaccatcactgctgcaggttgctattcttttagaatctttatgactccaggcaatgcagaatattccatttgttccatgctcattaaatcgttgtataattttgcccttttgaacattccaaataaaagcaccatttcgggaagttcccccagcaatacaatttaaaccacctggagcccaagaaagggaataaataacaccttcattacccggggatgtgtacactgctgttaatgtgtttatatcccagacttttatagtgccatcaaatgaagctgttgctaaaagattaggatcgtcaggtttgaatttgcagtcaaagatagtttccacatgtcccaagtctctaagaaaatcccacttcttagctcccatatcataaagtccaactccaccatccaagaaacaacacactgcatgaccaggaggaagagaaaatgcttgattctgtgttaaagttgggggtggaactgcttcgcttgttgaggatgtataatgatttttggttggagattggactgaaaacttttttcttggaggagaattaagtacatgtaagcagtgaaatcctgttttctttaatttaagattatcaataggtgttgttcttgaaacattccaaatgcgtaaaacacccacttgagaatagttctgcatggctgaggaggcctcaggaaacttacaatcatggtggaaggcaaagtagaagcaggcaccttctccagttataaacatcccaggagcactgggaacccaggctaagcactgtacagaagctgctgcactgggaagattaaatgttgttatgcaagaaagtgattcagaatctaccaggcgaattccataatgcaaattaaccactagaagataatcagtagatagtgggtcccattccaaggccgtaactggatcctcttcatctgtcccttcaagagattctggtctcaaaacatgtttctgatttttattacctggatgaaaaattgatagacttccatcaatatgaccaaacacaactttccccttttggtgtgtatgccatctgaacatacagatatcagacaagaagctatgagcatctttgtgtacaatcactccactatctggtcctgagatggtccaaatgaacagtgggcctctgtgggaaacaaatgccaccacatcctctgcattccagcaccaactaagagaagcagggatcccttttgtactgtcgagtttagcaatgactttttgttctgcaacattccaaatgatcactaaattatcagtactgccacttgcaaacagatcaggattatgtggacaccaagaaattgctgtgattgtttttttatgttcagacataattgcgtgaagtttgaattcattataacggtgatccaactgataaatatagatagccagggtcgcacaatatgcaaacctgtctccactggcagcacatacatccttgttccatggctgacatccagcagccagcaatcccacttgccttacctgggacatgtttgctctttgtagtccttcataccaatcatcttgctcaaaccaatttgaaatgtaagtcatccaagccatagaatgtttctactttaatcaaggcaattggaaactcggcatcagaatagtcagcacctaaagtaacaacaatgtgtttcaaccaaacaagatttaccaaaatctcccttgtgaaatgatgttcagtacaaaaggctagaactgcacaaatatttc

SEQ ID NO: 10830 - RNA, 5683 nt, Homo sapiens
  source 1..5683: mol_type = other RNA
ctgaatagctgggactacaggtacacaccaccacacccagctaatttttgtatttttagtagagacagggtttcaccatgttggccaggatggtctccatctaccgacctcaagatctgcccatctcggcctcctgaagtgctgggattacaggcaattttttttttttaataaaatggaatttaagcctgtaatgtctttttaaggaatcaaaagtggtcatgtgataaatatgatacatagatacataatatatattttttccagttttaagaagttttgttaagaaggttttaaaaatattttaaatgcaacaagtttaaagataataaaagccacaagtattctagttatatgagattattctttagtcaaacaaaaccatctatattataaatcttgtgaaacaacttgagtatcaaagtacttccagtatgcattaatttaataagtttcaaagtcagaattctagtccaactgaaatatctgtagtcacattatcaggcttttcatagcttcacacttttaaacaacattttaaaagttaaatcaacataatatatccaaaaattcaaccaatatctatttacaaacatttacttaaaactaattttcatcaaatcaattgtggtttttgttggtttgttttttgagacagagtttcgctctttgttgcccaggctggagtgcagtggtgcgatcttggctcactggaacctctgcctcccaggttcaagggattctcctgcctcagcttcccaagtaactgggattacaggtgcccgccaccatgcctggctaatttttgtatttttagtggagacagggttttaccatgctggccaggctggtcatgaactcctgacctcaggtgatccacctgccttggcctgccaaagtgctgagattacaggtgtgagccaccgtgcccggccaaataaattgtgttttaaataaagttaacataaattgactagagtatactgtgtaaattattgtacacattaatcaaaactaatatccatgcatgctgaatctcttaaaatagtcactttatcacctaatgcaagttttcatatatatattcgactgcattttgtgatttttacccgccaatttttttcaagcctatataacttacacctttacaatgggacagttaaacttcagataaaaaaactggtaacattttcttttttttaaaagtattttgaatgtgtatccatttattaatatttactaaacttataactgaaaacttttattaaaacagctaacgttagtggtttactatgcattttataaaggagaacgtaagtgtttgttaagttgaagatcactgtgcacaccttacatttcaacatttcaagatattcaatcattcaaatatccattaagtacttactgtatgtctagcactattctaggtgttgcacaatttaatatgtttcaatatttcaaccatatgatattttggtatcttttatgctgtgtgaaacttttatatgctttttagattattcagtcctttataatttaaatgtttcctccttcccaaacgtagctattactgtttataaaggaggcacctatttttcctttaaattatatatatatatatattttgaagttaatgactaaaattcactgctatttcccacctctcccaacctgcaatccttctcccaacctctggcacttgagcaacaaagattaaggtaatgctaacccatgaaagtttttctttaaaaaaaaaaatcaagcatggacaaaaatcttctatcagaatggattgagtcgtattccagtccctaaaggtgagaatggattcacctttgcccacatcaaagcatcattcaaggagatagcagatttcccgtcttcaaggaaaaacacagggccctggatttttaatcccgtaagacaagaaatgtgaatatcagaatgacttggaagatttgatccagtcacataatctggtccaataattcctttcagtgactcttcttttagtctctttaataaagttgcataaatcattctttgtgaatcagaagggggtgtatacggagagtcttctaatgatctgttggtggactgtgtgcaagctctccatgcatccaattcctcagaaagatattcaatttttaaaggtactgacacctcccgacgttttaatagctgacttgtgtactcataaagtgctggaacaatgctttggtactgtcttctgatagccagtaatgcaccaatgtaaccacataatatcagcaactcatttcgagcttcagtacacgtatgcaagagtaatttttcagtacgaatatagctcagtaggtcaagaacagggtatatggtatccaaagtccagtctgagctactgatgtattctttaacaaagctaataccaataggaagggctttttcaggttcttgacttaacaagtaatattttacagtttcaaatatattgtcatctgcacgggctgtctcagctaactgcatacattcttccactgtgggtagcttacacttatcatgaaggtcatttatctcttcagtacatcctgggtagaaagcacagagttttattaaatgtagttcattatcaggaatcatcagaagaagatcagctgccaaattcctgtatccaacacatggaaagcatactgaaatcatcatgcactttctcgccagtaattctaaggcatagtgggttgctggtgctgcagactctcctagtactgtgcccacacagactgccaactccagttcatttccgcgaatcaggtatgccatagcaagctcaatattatctatggcaagatggcaacatgcggctagtactgctcgaccatcttgaaaataccattctgccagttctttactgactttgtgcaggagttcattaaagtcttccttgtagatatcatcagaatatgaagctcctttaggcacggaaacatgtaagggctgcatatttccttcacaagcagcctgtgcaacaagcagagcttctttaagctgacctcttgacatgaaaaaatggactagctttttcacatcaccaatggctatgcagtatggaatgacatcatccttatcttcctggattaattggtcagctctcctctgcattaacttcttccagtatttcacagagactcctggtgcaattgacagggctttgtcccactctccaagttcaaccataagttcacagtatctctgaatttgtcctaatctcaagtggatttcagcagcttccttcagtctttcctctttagcaggtacaccaataccaccaccaaatttagacatcttgactgttgttagttcttgagcttcagatgttctaaatttaatcagatgtttcaagtgcattattcctttgcagtagttctgaggaagtaagctatcatcctgtccttttatcacagcaaccaagttccataaattgtcactgccacctggaggagataaacattctgagaaccatcttagttttttcacttgagaattagcagttagtttttctatttcctgtctaatatctcttgacactttaccacacagtagaggaggagtgcctggttctatagcataatcagtgttcccaataatttcttcccaagatctgtctgccagaatatttatttgtacaggagtgactaaggctgttaatgaccagagtctcactgtagagtcacgggagcaagaggccatagtgaaggggcgactgggatggcaggttaaaccatatacatctgcaccgtgatcatacacagtatccacacaagttccttctcgagtgtcccatacttttatagtatagtcccagctgccagatatgagcagatatggaatctcagtattccacattaatcctctcacaggtgcagtgtgtccattaagaatattgatgcaagcatcctgagtataatcccagattcgaacggtaccatcatcagaaccactgcaaagaattccctctctcagaggagaccatttaacatgaaacacttttgctgtatgcccactaaatactttcaatggttgatctgagctggtggctacataataaacacgaacatttgtgtcttcacagccagtggctatcatgtctttattgttttggctccaatcacaaccaaacactgcagctggatgtttatatttgtgtagcactttaccatcaattgttcgaataatacagaaaccatcactgctgcaggttgctattcttttagaatctttatgactccaggcaatgcagaatattccatttgttccatgctcattaaatcgttgtataattttgcccttttgaacattccaaataaaagcaccatttcgggaagttcccccagcaatacaatttaaaccacctggagcccaagaaagggaataaataacaccttcattacccggggatgtgtacactgctgttaatgtgtttatatcccagacttttatagtgccatcaaatgaagctgttgctaaaagattaggatcgtcaggtttgaatttgcagtcaaagatagtttccacatgtcccaagtctctaagaaaatcccacttcttagctcccatatcataaagtccaactccaccatccaagaaacaacacactgcatgaccaggaggaagagaaaatgcttgattctgtgttaaagttgggggtggaactgcttcgcttgttgaggatgtataatgatttttggttggagattggactgaaaacttttttcttggaggagaattaagtacatgtaagcagtgaaatcctgttttctttaatttaagattatcaataggtgttgttcttgaaacattccaaatgcgtaaaacacccacttgagaatctccagttataaacatcccaggagcactgggaacccaggctaagcactgtacagaagctgctgcactgggaagattaaatgttgttatgcaagaaagtgattcagaatctaccaggcgaattccataatgcaaattaaccactagaagataatcagtagatagtgggtcccattccaaggccgtaactggatcctcttcatctgtcccttcaagagattctggtctcaaaacatgtttctgatttttattacctggatgaaaaattgatagacttccatcaatatgaccaaacacaactttccccttttggtgtgtatgccatctgaacatacagatatcagacaagaagctatgagcatctttgtgtacaatcactccactatctggtcctgagatggtccaaatgaacagtgggcctctgtgggaaacaaatgccaccacatcctctgcattccagcaccaactaagagaagcagggatccctgataaatatagatagccagggtcgcacaatatgcaaacctgtctccactggcagcacatacatccttgttccatggctgacatccagcagccagcaatcccacttgccttacctgggacatgtttgctctttgtagtccttcataccaatcatcttgctcaaaccaatttgaaatgtaagtcatccaagccatagaatgtttctactttaatcaaggcaattggaaactcggcatcagaatagtcagcacctggaggaggaggcggctgcagcggcggacagcggaaggtgctgaagccggcgggcgcagctgcgaggcgagcaccaccaacg

SEQ ID NO: 10831 - RNA, 5900 nt, Homo sapiens
  source 1..5900: mol_type = other RNA
ctgaatagctgggactacaggtacacaccaccacacccagctaatttttgtatttttagtagagacagggtttcaccatgttggccaggatggtctccatctaccgacctcaagatctgcccatctcggcctcctgaagtgctgggattacaggcaattttttttttttaataaaatggaatttaagcctgtaatgtctttttaaggaatcaaaagtggtcatgtgataaatatgatacatagatacataatatatattttttccagttttaagaagttttgttaagaaggttttaaaaatattttaaatgcaacaagtttaaagataataaaagccacaagtattctagttatatgagattattctttagtcaaacaaaaccatctatattataaatcttgtgaaacaacttgagtatcaaagtacttccagtatgcattaatttaataagtttcaaagtcagaattctagtccaactgaaatatctgtagtcacattatcaggcttttcatagcttcacacttttaaacaacattttaaaagttaaatcaacataatatatccaaaaattcaaccaatatctatttacaaacatttacttaaaactaattttcatcaaatcaattgtggtttttgttggtttgttttttgagacagagtttcgctctttgttgcccaggctggagtgcagtggtgcgatcttggctcactggaacctctgcctcccaggttcaagggattctcctgcctcagcttcccaagtaactgggattacaggtgcccgccaccatgcctggctaatttttgtatttttagtggagacagggttttaccatgctggccaggctggtcatgaactcctgacctcaggtgatccacctgccttggcctgccaaagtgctgagattacaggtgtgagccaccgtgcccggccaaataaattgtgttttaaataaagttaacataaattgactagagtatactgtgtaaattattgtacacattaatcaaaactaatatccatgcatgctgaatctcttaaaatagtcactttatcacctaatgcaagttttcatatatatattcgactgcattttgtgatttttacccgccaatttttttcaagcctatataacttacacctttacaatgggacagttaaacttcagataaaaaaactggtaacattttcttttttttaaaagtattttgaatgtgtatccatttattaatatttactaaacttataactgaaaacttttattaaaacagctaacgttagtggtttactatgcattttataaaggagaacgtaagtgtttgttaagttgaagatcactgtgcacaccttacatttcaacatttcaagatattcaatcattcaaatatccattaagtacttactgtatgtctagcactattctaggtgttgcacaatttaatatgtttcaatatttcaaccatatgatattttggtatcttttatgctgtgtgaaacttttatatgctttttagattattcagtcctttataatttaaatgtttcctccttcccaaacgtagctattactgtttataaaggaggcacctatttttcctttaaattatatatatatatatattttgaagttaatgactaaaattcactgctatttcccacctctcccaacctgcaatccttctcccaacctctggcacttgagcaacaaagattaaggtaatgctaacccatgaaagtttttctttaaaaaaaaaaatcaagcatggacaaaaatcttctatcagaatggattgagtcgtattccagtccctaaaggtgagaatggattcacctttgcccacatcaaagcatcattcaaggagatagcagatttcccgtcttcaaggaaaaacacagggccctggatttttaatcccgtaagacaagaaatgtgaatatcagaatgacttggaagatttgatccagtcacataatctggtccaataattcctttcagtgactcttcttttagtctctttaataaagttgcataaatcattctttgtgaatcagaagggggtgtatacggagagtcttctaatgatctgttggtggactgtgtgcaagctctccatgcatccaattcctcagaaagatattcaatttttaaaggtactgacacctcccgacgttttaatagctgacttgtgtactcataaagtgctggaacaatgctttggtactgtcttctgatagccagtaatgcaccaatgtaaccacataatatcagcaactcatttcgagcttcagtacacgtatgcaagagtaatttttcagtacgaatatagctcagtaggtcaagaacagggtatatggtatccaaagtccagtctgagctactgatgtattctttaacaaagctaataccaataggaagggctttttcaggttcttgacttaacaagtaatattttacagtttcaaatatattgtcatctgcacgggctgtctcagctaactgcatacattcttccactgtgggtagcttacacttatcatgaaggtcatttatctcttcagtacatcctgggtagaaagcacagagttttattaaatgtagttcattatcaggaatcatcagaagaagatcagctgccaaattcctgtatccaacacatggaaagcatactgaaatcatcatgcactttctcgccagtaattctaaggcatagtgggttgctggtgctgcagactctcctagtactgtgcccacacagactgccaactccagttcatttccgcgaatcaggtatgccatagcaagctcaatattatctatggcaagatggcaacatgcggctagtactgctcgaccatcttgaaaataccattctgccagttctttactgactttgtgcaggagttcattaaagtcttccttgtagatatcatcagaatatgaagctcctttaggcacggaaacatgtaagggctgcatatttccttcacaagcagcctgtgcaacaagcagagcttctttaagctgacctcttgacatgaaaaaatggactagctttttcacatcaccaatggctatgcagtatggaatgacatcatccttatcttcctggattaattggtcagctctcctctgcattaacttcttccagtatttcacagagactcctggtgcaattgacagggctttgtcccactctccaagttcaaccataagttcacagtatctctgaatttgtcctaatctcaagtggatttcagcagcttccttcagtctttcctctttagcaggtacaccaataccaccaccaaatttagacatcttgactgttgttagttcttgagcttcagatgttctaaatttaatcagatgtttcaagtgcattattcctttgcagtagttctgaggaagtaagctatcatcctgtccttttatcacagcaaccaagttccataaattgtcactgccacctggaggagataaacattctgagaaccatcttagttttttcacttgagaattagcagttagtttttctatttcctgtctaatatctcttgacactttaccacacagtagaggaggagtgcctggttctatagcataatcagtgttcccaataatttcttcccaagatctgtctgccagaatatttatttgtacaggagtgactaaggctgttaatgaccagagtctcactgtagagtcacgggagcaagaggccatagtgaaggggcgactgggatggcaggttaaaccatatacatctgcaccgtgatcatacacagtatccacacaagttccttctcgagtgtcccatacttttatagtatagtcccagctgccagatatgagcagatatggaatctcagtattccacattaatcctctcacaggtgcagtgtgtccattaagaatattgatgcaagcatcctgagtataatcccagattcgaacggtaccatcatcagaaccactgcaaagaattccctctctcagaggagaccatttaacatgaaacacttttgctgtatgcccactaaatactttcaatggttgatctgagctggtggctacataataaacacgaacatttgtgtcttcacagccagtggctatcatgtctttattgttttggctccaatcacaaccaaacactgcagctggatgtttatatttgtgtagcactttaccatcaattgttcgaataatacagaaaccatcactgctgcaggttgctattcttttagaatctttatgactccaggcaatgcagaatattccatttgttccatgctcattaaatcgttgtataattttgcccttttgaacattccaaataaaagcaccatttcgggaagttcccccagcaatacaatttaaaccacctggagcccaagaaagggaataaataacaccttcattacccggggatgtgtacactgctgttaatgtgtttatatcccagacttttatagtgccatcaaatgaagctgttgctaaaagattaggatcgtcaggtttgaatttgcagtcaaagatagtttccacatgtcccaagtctctaagaaaatcccacttcttagctcccatatcataaagtccaactccaccatccaagaaacaacacactgcatgaccaggaggaagagaaaatgcttgattctgtgttaaagttgggggtggaactgcttcgcttgttgaggatgtataatgatttttggttggagattggactgaaaacttttttcttggaggagaattaagtacatgtaagcagtgaaatcctgttttctttaatttaagattatcaataggtgttgttcttgaaacattccaaatgcgtaaaacacccacttgagaatctccagttataaacatcccaggagcactgggaacccaggctaagcactgtacagaagctgctgcactgggaagattaaatgttgttatgcaagaaagtgattcagaatctaccaggcgaattccataatgcaaattaaccactagaagataatcagtagatagtgggtcccattccaaggccgtaactggatcctcttcatctgtcccttcaagagattctggtctcaaaacatgtttctgatttttattacctggatgaaaaattgatagacttccatcaatatgaccaaacacaactttccccttttggtgtgtatgccatctgaacatacagatatcagacaagaagctatgagcatctttgtgtacaatcactccactatctggtcctgagatggtccaaatgaacagtgggcctctgtgggaaacaaatgccaccacatcctctgcattccagcaccaactaagagaagcagggatcccttttgtactgtcgagtttagcaatgactttttgttctgcaacattccaaatgatcactaaattatcagtactgccacttgcaaacagatcaggattatgtggacaccaagaaattgctgtgattgtttttttatgttcagacataattgcgtgaagtttgaattcattataacggtgatccaactgataaatatagatagccagggtcgcacaatatgcaaacctgtctccactggcagcacatacatccttgttccatggctgacatccagcagccagcaatcccacttgccttacctgggacatgtttgcctggaggaggaggcggctgcagcggcggacagcggaaggtgctgaagccggcgggcgcagctgcgaggcgagcaccaccaacgcgcggaccctccccgccctccccgcctgctcgctcagggcgcccgggggcggggcggccgggcccgcgggctccgaggggcgggaagcgtgctccgcaagccccagcgcggagccacgatggaaggcgccgcgagcccgatctccagggtctgccc

SEQ ID NO: 10832 - RNA, 5883 nt, Homo sapiens
  source 1..5883: mol_type = other RNA
ctgaatagctgggactacaggtacacaccaccacacccagctaatttttgtatttttagtagagacagggtttcaccatgttggccaggatggtctccatctaccgacctcaagatctgcccatctcggcctcctgaagtgctgggattacaggcaattttttttttttaataaaatggaatttaagcctgtaatgtctttttaaggaatcaaaagtggtcatgtgataaatatgatacatagatacataatatatattttttccagttttaagaagttttgttaagaaggttttaaaaatattttaaatgcaacaagtttaaagataataaaagccacaagtattctagttatatgagattattctttagtcaaacaaaaccatctatattataaatcttgtgaaacaacttgagtatcaaagtacttccagtatgcattaatttaataagtttcaaagtcagaattctagtccaactgaaatatctgtagtcacattatcaggcttttcatagcttcacacttttaaacaacattttaaaagttaaatcaacataatatatccaaaaattcaaccaatatctatttacaaacatttacttaaaactaattttcatcaaatcaattgtggtttttgttggtttgttttttgagacagagtttcgctctttgttgcccaggctggagtgcagtggtgcgatcttggctcactggaacctctgcctcccaggttcaagggattctcctgcctcagcttcccaagtaactgggattacaggtgcccgccaccatgcctggctaatttttgtatttttagtggagacagggttttaccatgctggccaggctggtcatgaactcctgacctcaggtgatccacctgccttggcctgccaaagtgctgagattacaggtgtgagccaccgtgcccggccaaataaattgtgttttaaataaagttaacataaattgactagagtatactgtgtaaattattgtacacattaatcaaaactaatatccatgcatgctgaatctcttaaaatagtcactttatcacctaatgcaagttttcatatatatattcgactgcattttgtgatttttacccgccaatttttttcaagcctatataacttacacctttacaatgggacagttaaacttcagataaaaaaactggtaacattttcttttttttaaaagtattttgaatgtgtatccatttattaatatttactaaacttataactgaaaacttttattaaaacagctaacgttagtggtttactatgcattttataaaggagaacgtaagtgtttgttaagttgaagatcactgtgcacaccttacatttcaacatttcaagatattcaatcattcaaatatccattaagtacttactgtatgtctagcactattctaggtgttgcacaatttaatatgtttcaatatttcaaccatatgatattttggtatcttttatgctgtgtgaaacttttatatgctttttagattattcagtcctttataatttaaatgtttcctccttcccaaacgtagctattactgtttataaaggaggcacctatttttcctttaaattatatatatatatatattttgaagttaatgactaaaattcactgctatttcccacctctcccaacctgcaatccttctcccaacctctggcacttgagcaacaaagattaaggtaatgctaacccatgaaagtttttctttaaaaaaaaaaatcaagcatggacaaaaatcttctatcagaatggattgagtcgtattccagtccctaaaggtgagaatggattcacctttgcccacatcaaagcatcattcaaggagatagcagatttcccgtcttcaaggaaaaacacagggccctggatttttaatcccgtaagacaagaaatgtgaatatcagaatgacttggaagatttgatccagtcacataatctggtccaataattcctttcagtgactcttcttttagtctctttaataaagttgcataaatcattctttgtgaatcagaagggggtgtatacggagagtcttctaatgatctgttggtggactgtgtgcaagctctccatgcatccaattcctcagaaagatattcaatttttaaaggtactgacacctcccgacgttttaatagctgacttgtgtactcataaagtgctggaacaatgctttggtactgtcttctgatagccagtaatgcaccaatgtaaccacataatatcagcaactcatttcgagcttcagtacacgtatgcaagagtaatttttcagtacgaatatagctcagtaggtcaagaacagggtatatggtatccaaagtccagtctgagctactgatgtattctttaacaaagctaataccaataggaagggctttttcaggttcttgacttaacaagtaatattttacagtttcaaatatattgtcatctgcacgggctgtctcagctaactgcatacattcttccactgtgggtagcttacacttatcatgaaggtcatttatctcttcagtacatcctgggtagaaagcacagagttttattaaatgtagttcattatcaggaatcatcagaagaagatcagctgccaaattcctgtatccaacacatggaaagcatactgaaatcatcatgcactttctcgccagtaattctaaggcatagtgggttgctggtgctgcagactctcctagtactgtgcccacacagactgccaactccagttcatttccgcgaatcaggtatgccatagcaagctcaatattatctatggcaagatggcaacatgcggctagtactgctcgaccatcttgaaaataccattctgccagttctttactgactttgtgcaggagttcattaaagtcttccttgtagatatcatcagaatatgaagctcctttaggcacggaaacatgtaagggctgcatatttccttcacaagcagcctgtgcaacaagcagagcttctttaagctgacctcttgacatgaaaaaatggactagctttttcacatcaccaatggctatgcagtatggaatgacatcatccttatcttcctggattaattggtcagctctcctctgcattaacttcttccagtatttcacagagactcctggtgcaattgacagggctttgtcccactctccaagttcaaccataagttcacagtatctctgaatttgtcctaatctcaagtggatttcagcagcttccttcagtctttcctctttagcaggtacaccaataccaccaccaaatttagacatcttgactgttgttagttcttgagcttcagatgttctaaatttaatcagatgtttcaagtgcattattcctttgcagtagttctgaggaagtaagctatcatcctgtccttttatcacagcaaccaagttccataaattgtcactgccacctggaggagataaacattctgagaaccatcttagttttttcacttgagaattagcagttagtttttctatttcctgtctaatatctcttgacactttaccacacagtagaggaggagtgcctggttctatagcataatcagtgttcccaataatttcttcccaagatctgtctgccagaatatttatttgtacaggagtgactaaggctgttaatgaccagagtctcactgtagagtcacgggagcaagaggccatagtgaaggggcgactgggatggcaggttaaaccatatacatctgcaccgtgatcatacacagtatccacacaagttccttctcgagtgtcccatacttttatagtatagtcccagctgccagatatgagcagatatggaatctcagtattccacattaatcctctcacaggtgcagtgtgtccattaagaatattgatgcaagcatcctgagtataatcccagattcgaacggtaccatcatcagaaccactgcaaagaattccctctctcagaggagaccatttaacatgaaacacttttgctgtatgcccactaaatactttcaatggttgatctgagctggtggctacataataaacacgaacatttgtgtcttcacagccagtggctatcatgtctttattgttttggctccaatcacaaccaaacactgcagctggatgtttatatttgtgtagcactttaccatcaattgttcgaataatacagaaaccatcactgctgcaggttgctattcttttagaatctttatgactccaggcaatgcagaatattccatttgttccatgctcattaaatcgttgtataattttgcccttttgaacattccaaataaaagcaccatttcgggaagttcccccagcaatacaatttaaaccacctggagcccaagaaagggaataaataacaccttcattacccggggatgtgtacactgctgttaatgtgtttatatcccagacttttatagtgccatcaaatgaagctgttgctaaaagattaggatcgtcaggtttgaatttgcagtcaaagatagtttccacatgtcccaagtctctaagaaaatcccacttcttagctcccatatcataaagtccaactccaccatccaagaaacaacacactgcatgaccaggaggaagagaaaatgcttgattctgtgttaaagttgggggtggaactgcttcgcttgttgaggatgtataatgatttttggttggagattggactgaaaacttttttcttggaggagaattaagtacatgtaagcagtgaaatcctgttttctttaatttaagattatcaataggtgttgttcttgaaacattccaaatgcgtaaaacacccacttgagaatctccagttataaacatcccaggagcactgggaacccaggctaagcactgtacagaagctgctgcactgggaagattaaatgttgttatgcaagaaagtgattcagaatctaccaggcgaattccataatgcaaattaaccactagaagataatcagtagatagtgggtcccattccaaggccgtaactggatcctcttcatctgtcccttcaagagattctggtctcaaaacatgtttctgatttttattacctggatgaaaaattgatagacttccatcaatatgaccaaacacaactttccccttttggtgtgtatgccatctgaacatacagatatcagacaagaagctatgagcatctttgtgtacaatcactccactatctggtcctgagatggtccaaatgaacagtgggcctctgtgggaaacaaatgccaccacatcctctgcattccagcaccaactaagagaagcagggatcccttttgtactgtcgagtttagcaatgactttttgttctgcaacattccaaatgatcactaaattatcagtactgccacttgcaaacagatcaggattatgtggacaccaagaaattgctgtgattgtttttttatgttcagacataattgcgtgaagtttgaattcattataacggtgatccaactgataaatatagatagccagggtcgcacaatatgcaaacctgtctccactggcagcacatacatccttgttccatggctgacatccagcagccagcaatcccacttgccttacctgggacatgtttgctctttgtagtccttcataccaatcatcttgctcaaaccaatttgaaatgtaagtcatccaagccatagaatgtttctactttaatcaaggcaattggaaactcggcatcagaatagtcagcacctaaagtaacaacaatgtgtttcaaccaaacaagatttaccaaaatctcccttgtgaaatgatgttcagtacaaaaggctagaactgcacaaatatttc

SEQ ID NO: 10833 - RNA, 6023 nt, Homo sapiens
  source 1..6023: mol_type = other RNA
ctgaatagctgggactacaggtacacaccaccacacccagctaatttttgtatttttagtagagacagggtttcaccatgttggccaggatggtctccatctaccgacctcaagatctgcccatctcggcctcctgaagtgctgggattacaggcaattttttttttttaataaaatggaatttaagcctgtaatgtctttttaaggaatcaaaagtggtcatgtgataaatatgatacatagatacataatatatattttttccagttttaagaagttttgttaagaaggttttaaaaatattttaaatgcaacaagtttaaagataataaaagccacaagtattctagttatatgagattattctttagtcaaacaaaaccatctatattataaatcttgtgaaacaacttgagtatcaaagtacttccagtatgcattaatttaataagtttcaaagtcagaattctagtccaactgaaatatctgtagtcacattatcaggcttttcatagcttcacacttttaaacaacattttaaaagttaaatcaacataatatatccaaaaattcaaccaatatctatttacaaacatttacttaaaactaattttcatcaaatcaattgtggtttttgttggtttgttttttgagacagagtttcgctctttgttgcccaggctggagtgcagtggtgcgatcttggctcactggaacctctgcctcccaggttcaagggattctcctgcctcagcttcccaagtaactgggattacaggtgcccgccaccatgcctggctaatttttgtatttttagtggagacagggttttaccatgctggccaggctggtcatgaactcctgacctcaggtgatccacctgccttggcctgccaaagtgctgagattacaggtgtgagccaccgtgcccggccaaataaattgtgttttaaataaagttaacataaattgactagagtatactgtgtaaattattgtacacattaatcaaaactaatatccatgcatgctgaatctcttaaaatagtcactttatcacctaatgcaagttttcatatatatattcgactgcattttgtgatttttacccgccaatttttttcaagcctatataacttacacctttacaatgggacagttaaacttcagataaaaaaactggtaacattttcttttttttaaaagtattttgaatgtgtatccatttattaatatttactaaacttataactgaaaacttttattaaaacagctaacgttagtggtttactatgcattttataaaggagaacgtaagtgtttgttaagttgaagatcactgtgcacaccttacatttcaacatttcaagatattcaatcattcaaatatccattaagtacttactgtatgtctagcactattctaggtgttgcacaatttaatatgtttcaatatttcaaccatatgatattttggtatcttttatgctgtgtgaaacttttatatgctttttagattattcagtcctttataatttaaatgtttcctccttcccaaacgtagctattactgtttataaaggaggcacctatttttcctttaaattatatatatatatatattttgaagttaatgactaaaattcactgctatttcccacctctcccaacctgcaatccttctcccaacctctggcacttgagcaacaaagattaaggtaatgctaacccatgaaagtttttctttaaaaaaaaaaatcaagcatggacaaaaatcttctatcagaatggattgagtcgtattccagtccctaaaggtgagaatggattcacctttgcccacatcaaagcatcattcaaggagatagcagatttcccgtcttcaaggaaaaacacagggccctggatttttaatcccgtaagacaagaaatgtgaatatcagaatgacttggaagatttgatccagtcacataatctggtccaataattcctttcagtgactcttcttttagtctctttaataaagttgcataaatcattctttgtgaatcagaagggggtgtatacggagagtcttctaatgatctgttggtggactgtgtgcaagctctccatgcatccaattcctcagaaagatattcaatttttaaaggtactgacacctcccgacgttttaatagctgacttgtgtactcataaagtgctggaacaatgctttggtactgtcttctgatagccagtaatgcaccaatgtaaccacataatatcagcaactcatttcgagcttcagtacacgtatgcaagagtaatttttcagtacgaatatagctcagtaggtcaagaacagggtatatggtatccaaagtccagtctgagctactgatgtattctttaacaaagctaataccaataggaagggctttttcaggttcttgacttaacaagtaatattttacagtttcaaatatattgtcatctgcacgggctgtctcagctaactgcatacattcttccactgtgggtagcttacacttatcatgaaggtcatttatctcttcagtacatcctgggtagaaagcacagagttttattaaatgtagttcattatcaggaatcatcagaagaagatcagctgccaaattcctgtatccaacacatggaaagcatactgaaatcatcatgcactttctcgccagtaattctaaggcatagtgggttgctggtgctgcagactctcctagtactgtgcccacacagactgccaactccagttcatttccgcgaatcaggtatgccatagcaagctcaatattatctatggcaagatggcaacatgcggctagtactgctcgaccatcttgaaaataccattctgccagttctttactgactttgtgcaggagttcattaaagtcttccttgtagatatcatcagaatatgaagctcctttaggcacggaaacatgtaagggctgcatatttccttcacaagcagcctgtgcaacaagcagagcttctttaagctgacctcttgacatgaaaaaatggactagctttttcacatcaccaatggctatgcagtatggaatgacatcatccttatcttcctggattaattggtcagctctcctctgcattaacttcttccagtatttcacagagactcctggtgcaattgacagggctttgtcccactctccaagttcaaccataagttcacagtatctctgaatttgtcctaatctcaagtggatttcagcagcttccttcagtctttcctctttagcaggtacaccaataccaccaccaaatttagacatcttgactgttgttagttcttgagcttcagatgttctaaatttaatcagatgtttcaagtgcattattcctttgcagtagttctgaggaagtaagctatcatcctgtccttttatcacagcaaccaagttccataaattgtcactgccacctggaggagataaacattctgagaaccatcttagttttttcacttgagaattagcagttagtttttctatttcctgtctaatatctcttgacactttaccacacagtagaggaggagtgcctggttctatagcataatcagtgttcccaataatttcttcccaagatctgtctgccagaatatttatttgtacaggagtgactaaggctgttaatgaccagagtctcactgtagagtcacgggagcaagaggccatagtgaaggggcgactgggatggcaggttaaaccatatacatctgcaccgtgatcatacacagtatccacacaagttccttctcgagtgtcccatacttttatagtatagtcccagctgccagatatgagcagatatggaatctcagtattccacattaatcctctcacaggtgcagtgtgtccattaagaatattgatgcaagcatcctgagtataatcccagattcgaacggtaccatcatcagaaccactgcaaagaattccctctctcagaggagaccatttaacatgaaacacttttgctgtatgcccactaaatactttcaatggttgatctgagctggtggctacataataaacacgaacatttgtgtcttcacagccagtggctatcatgtctttattgttttggctccaatcacaaccaaacactgcagctggatgtttatatttgtgtagcactttaccatcaattgttcgaataatacagaaaccatcactgctgcaggttgctattcttttagaatctttatgactccaggcaatgcagaatattccatttgttccatgctcattaaatcgttgtataattttgcccttttgaacattccaaataaaagcaccatttcgggaagttcccccagcaatacaatttaaaccacctggagcccaagaaagggaataaataacaccttcattacccggggatgtgtacactgctgttaatgtgtttatatcccagacttttatagtgccatcaaatgaagctgttgctaaaagattaggatcgtcaggtttgaatttgcagtcaaagatagtttccacatgtcccaagtctctaagaaaatcccacttcttagctcccatatcataaagtccaactccaccatccaagaaacaacacactgcatgaccaggaggaagagaaaatgcttgattctgtgttaaagttgggggtggaactgcttcgcttgttgaggatgtataatgatttttggttggagattggactgaaaacttttttcttggaggagaattaagtacatgtaagcagtgaaatcctgttttctttaatttaagattatcaataggtgttgttcttgaaacattccaaatgcgtaaaacacccacttgagaatctccagttataaacatcccaggagcactgggaacccaggctaagcactgtacagaagctgctgcactgggaagattaaatgttgttatgcaagaaagtgattcagaatctaccaggcgaattccataatgcaaattaaccactagaagataatcagtagatagtgggtcccattccaaggccgtaactggatcctcttcatctgtcccttcaagagattctggtctcaaaacatgtttctgatttttattacctggatgaaaaattgatagacttccatcaatatgaccaaacacaactttccccttttggtgtgtatgccatctgaacatacagatatcagacaagaagctatgagcatctttgtgtacaatcactccactatctggtcctgagatggtccaaatgaacagtgggcctctgtgggaaacaaatgccaccacatcctctgcattccagcaccaactaagagaagcagggatcccttttgtactgtcgagtttagcaatgactttttgttctgcaacattccaaatgatcactaaattatcagtactgccacttgcaaacagatcaggattatgtggacaccaagaaattgctgtgattgtttttttatgttcagacataattgcgtgaagtttgaattcattataacggtgatccaactgataaatatagatagccagggtcgcacaatatgcaaacctgtctccactggcagcacatacatccttgttccatggctgacatccagcagccagcaatcccacttgccttacctgggacatgtttgctctttgtagtccttcataccaatcatcttgctcaaaccaatttgaaatgtaagtcatccaagccatagaatgtttctactttaatcaaggcaattggaaactcggcatcagaatagtcagcacctggaggaggaggcggctgcagcggcggacagcggaaggtgctgaagccggcgggcgcagctgcgaggcgagcaccaccaacgcgcggaccctccccgccctccccgcctgctcgctcagggcgcccgggggcggggcggccgggcccgcgggctccgaggggcgggaagcgtgctccgcaagccccagcgcggagccacgatggaaggcgccgcgagcccgatctccagggtctgccc

SEQ ID NO: 10834 - RNA, 5664 nt, Homo sapiens
  source 1..5664: mol_type = other RNA
ctgaatagctgggactacaggtacacaccaccacacccagctaatttttgtatttttagtagagacagggtttcaccatgttggccaggatggtctccatctaccgacctcaagatctgcccatctcggcctcctgaagtgctgggattacaggcaattttttttttttaataaaatggaatttaagcctgtaatgtctttttaaggaatcaaaagtggtcatgtgataaatatgatacatagatacataatatatattttttccagttttaagaagttttgttaagaaggttttaaaaatattttaaatgcaacaagtttaaagataataaaagccacaagtattctagttatatgagattattctttagtcaaacaaaaccatctatattataaatcttgtgaaacaacttgagtatcaaagtacttccagtatgcattaatttaataagtttcaaagtcagaattctagtccaactgaaatatctgtagtcacattatcaggcttttcatagcttcacacttttaaacaacattttaaaagttaaatcaacataatatatccaaaaattcaaccaatatctatttacaaacatttacttaaaactaattttcatcaaatcaattgtggtttttgttggtttgttttttgagacagagtttcgctctttgttgcccaggctggagtgcagtggtgcgatcttggctcactggaacctctgcctcccaggttcaagggattctcctgcctcagcttcccaagtaactgggattacaggtgcccgccaccatgcctggctaatttttgtatttttagtggagacagggttttaccatgctggccaggctggtcatgaactcctgacctcaggtgatccacctgccttggcctgccaaagtgctgagattacaggtgtgagccaccgtgcccggccaaataaattgtgttttaaataaagttaacataaattgactagagtatactgtgtaaattattgtacacattaatcaaaactaatatccatgcatgctgaatctcttaaaatagtcactttatcacctaatgcaagttttcatatatatattcgactgcattttgtgatttttacccgccaatttttttcaagcctatataacttacacctttacaatgggacagttaaacttcagataaaaaaactggtaacattttcttttttttaaaagtattttgaatgtgtatccatttattaatatttactaaacttataactgaaaacttttattaaaacagctaacgttagtggtttactatgcattttataaaggagaacgtaagtgtttgttaagttgaagatcactgtgcacaccttacatttcaacatttcaagatattcaatcattcaaatatccattaagtacttactgtatgtctagcactattctaggtgttgcacaatttaatatgtttcaatatttcaaccatatgatattttggtatcttttatgctgtgtgaaacttttatatgctttttagattattcagtcctttataatttaaatgtttcctccttcccaaacgtagctattactgtttataaaggaggcacctatttttcctttaaattatatatatatatatattttgaagttaatgactaaaattcactgctatttcccacctctcccaacctgcaatccttctcccaacctctggcacttgagcaacaaagattaaggtaatgctaacccatgaaagtttttctttaaaaaaaaaaatcaagcatggacaaaaatcttctatcagaatggattgagtcgtattccagtccctaaaggtgagaatggattcacctttgcccacatcaaagcatcattcaaggagatagcagatttcccgtcttcaaggaaaaacacagggccctggatttttaatcccgtaagacaagaaatgtgaatatcagaatgacttggaagatttgatccagtcacataatctggtccaataattcctttcagtgactcttcttttagtctctttaataaagttgcataaatcattctttgtgaatcagaagggggtgtatacggagagtcttctaatgatctgttggtggactgtgtgcaagctctccatgcatccaattcctcagaaagatattcaatttttaaaggtactgacacctcccgacgttttaatagctgacttgtgtactcataaagtgctggaacaatgctttggtactgtcttctgatagccagtaatgcaccaatgtaaccacataatatcagcaactcatttcgagcttcagtacacgtatgcaagagtaatttttcagtacgaatatagctcagtaggtcaagaacagggtatatggtatccaaagtccagtctgagctactgatgtattctttaacaaagctaataccaataggaagggctttttcaggttcttgacttaacaagtaatattttacagtttcaaatatattgtcatctgcacgggctgtctcagctaactgcatacattcttccactgtgggtagcttacacttatcatgaaggtcatttatctcttcagtacatcctgggtagaaagcacagagttttattaaatgtagttcattatcaggaatcatcagaagaagatcagctgccaaattcctgtatccaacacatggaaagcatactgaaatcatcatgcactttctcgccagtaattctaaggcatagtgggttgctggtgctgcagactctcctagtactgtgcccacacagactgccaactccagttcatttccgcgaatcaggtatgccatagcaagctcaatattatctatggcaagatggcaacatgcggctagtactgctcgaccatcttgaaaataccattctgccagttctttactgactttgtgcaggagttcattaaagtcttccttgtagatatcatcagaatatgaagctcctttaggcacggaaacatgtaagggctgcatatttccttcacaagcagcctgtgcaacaagcagagcttctttaagctgacctcttgacatgaaaaaatggactagctttttcacatcaccaatggctatgcagtatggaatgacatcatccttatcttcctggattaattggtcagctctcctctgcattaacttcttccagtatttcacagagactcctggtgcaattgacagggctttgtcccactctccaagttcaaccataagttcacagtatctctgaatttgtcctaatctcaagtggatttcagcagcttccttcagtctttcctctttagcaggtacaccaataccaccaccaaatttagacatcttgactgttgttagttcttgagcttcagatgttctaaatttaatcagatgtttcaagtgcattattcctttgcagtagttctgaggaagtaagctatcatcctgtccttttatcacagcaaccaagttccataaattgtcactgccacctggaggagataaacattctgagaaccatcttagttttttcacttgagaattagcagttagtttttctatttcctgtctaatatctcttgacactttaccacacagtagaggaggagtgcctggttctatagcataatcagtgttcccaataatttcttcccaagatctgtctgccagaatatttatttgtacaggagtgactaaggctgttaatgaccagagtctcactgtagagtcacgggagcaagaggccatagtgaaggggcgactgggatggcaggttaaaccatatacatctgcaccgtgatcatacacagtatccacacaagttccttctcgagtgtcccatacttttatagtatagtcccagctgccagatatgagcagatatggaatctcagtattccacattaatcctctcacaggtgcagtgtgtccattaagaatattgatgcaagcatcctgagtataatcccagattcgaacggtattattgttttggctccaatcacaaccaaacactgcagctggatgtttatatttgtgtagcactttaccatcaattgttcgaataatacagaaaccatcactgctgcaggttgctattcttttagaatctttatgactccaggcaatgcagaatattccatttgttccatgctcattaaatcgttgtataattttgcccttttgaacattccaaataaaagcaccatttcgggaagttcccccagcaatacaatttaaaccacctggagcccaagaaagggaataaataacaccttcattacccggggatgtgtacactgctgttaatgtgtttatatcccagacttttatagtgccatcaaatgaagctgttgctaaaagattaggatcgtcaggtttgaatttgcagtcaaagatagtttccacatgtcccaagtctctaagaaaatcccacttcttagctcccatatcataaagtccaactccaccatccaagaaacaacacactgcatgaccaggaggaagagaaaatgcttgattctgtgttaaagttgggggtggaactgcttcgcttgttgaggatgtataatgatttttggttggagattggactgaaaacttttttcttggaggagaattaagtacatgtaagcagtgaaatcctgttttctttaatttaagattatcaataggtgttgttcttgaaacattccaaatgcgtaaaacacccacttgagaatagttctgcatggctgaggaggcctcaggaaacttacaatcatggtggaaggcaaagtagaagcaggcaccttctccagttataaacatcccaggagcactgggaacccaggctaagcactgtacagaagctgctgcactgggaagattaaatgttgttatgcaagaaagtgattcagaatctaccaggcgaattccataatgcaaattaaccactagaagataatcagtagatagtgggtcccattccaaggccgtaactggatcctcttcatctgtcccttcaagagattctggtctcaaaacatgtttctgatttttattacctggatgaaaaattgatagacttccatcaatatgaccaaacacaactttccccttttggtgtgtatgccatctgaacatacagatatcagacaagaagctatgagcatctttgtgtacaatcactccactatctggtcctgagatggtccaaatgaacagtgggcctctgtgggaaacaaatgccaccacatcctctgcattccagcaccaactaagagaagcagggatcccttttgtactgtcgagtttagcaatgactttttgttctgcaacattccaaatgatcactaaattatcagtactgccacttgcaaacagatcaggattatgtggacaccaagaaattgctgtgattgtttttttatgttcagacataattgcgtgaagtttgaattcattataacggtgatccaactgataaatatagatagccagggtcgcacaatatgcaaacctgtctccactggcagcacatacatccttgttccatggctgacatccagcagccagcaatcccacttgccttacctgggacatgtttgcctggaggaggaggcggctgcagcggcggacagcggaaggtgctgaagccggcgggcgcagctgcgaggcgagcaccaccaacgcgcggaccctccc

SEQ ID NO: 10835 - RNA, 5735 nt, Homo sapiens
  source 1..5735: mol_type = other RNA
ctgaatagctgggactacaggtacacaccaccacacccagctaatttttgtatttttagtagagacagggtttcaccatgttggccaggatggtctccatctaccgacctcaagatctgcccatctcggcctcctgaagtgctgggattacaggcaattttttttttttaataaaatggaatttaagcctgtaatgtctttttaaggaatcaaaagtggtcatgtgataaatatgatacatagatacataatatatattttttccagttttaagaagttttgttaagaaggttttaaaaatattttaaatgcaacaagtttaaagataataaaagccacaagtattctagttatatgagattattctttagtcaaacaaaaccatctatattataaatcttgtgaaacaacttgagtatcaaagtacttccagtatgcattaatttaataagtttcaaagtcagaattctagtccaactgaaatatctgtagtcacattatcaggcttttcatagcttcacacttttaaacaacattttaaaagttaaatcaacataatatatccaaaaattcaaccaatatctatttacaaacatttacttaaaactaattttcatcaaatcaattgtggtttttgttggtttgttttttgagacagagtttcgctctttgttgcccaggctggagtgcagtggtgcgatcttggctcactggaacctctgcctcccaggttcaagggattctcctgcctcagcttcccaagtaactgggattacaggtgcccgccaccatgcctggctaatttttgtatttttagtggagacagggttttaccatgctggccaggctggtcatgaactcctgacctcaggtgatccacctgccttggcctgccaaagtgctgagattacaggtgtgagccaccgtgcccggccaaataaattgtgttttaaataaagttaacataaattgactagagtatactgtgtaaattattgtacacattaatcaaaactaatatccatgcatgctgaatctcttaaaatagtcactttatcacctaatgcaagttttcatatatatattcgactgcattttgtgatttttacccgccaatttttttcaagcctatataacttacacctttacaatgggacagttaaacttcagataaaaaaactggtaacattttcttttttttaaaagtattttgaatgtgtatccatttattaatatttactaaacttataactgaaaacttttattaaaacagctaacgttagtggtttactatgcattttataaaggagaacgtaagtgtttgttaagttgaagatcactgtgcacaccttacatttcaacatttcaagatattcaatcattcaaatatccattaagtacttactgtatgtctagcactattctaggtgttgcacaatttaatatgtttcaatatttcaaccatatgatattttggtatcttttatgctgtgtgaaacttttatatgctttttagattattcagtcctttataatttaaatgtttcctccttcccaaacgtagctattactgtttataaaggaggcacctatttttcctttaaattatatatatatatatattttgaagttaatgactaaaattcactgctatttcccacctctcccaacctgcaatccttctcccaacctctggcacttgagcaacaaagattaaggtaatgctaacccatgaaagtttttctttaaaaaaaaaaatcaagcatggacaaaaatcttctatcagaatggattgagtcgtattccagtccctaaaggtgagaatggattcacctttgcccacatcaaagcatcattcaaggagatagcagatttcccgtcttcaaggaaaaacacagggccctggatttttaatcccgtaagacaagaaatgtgaatatcagaatgacttggaagatttgatccagtcacataatctggtccaataattcctttcagtgactcttcttttagtctctttaataaagttgcataaatcattctttgtgaatcagaagggggtgtatacggagagtcttctaatgatctgttggtggactgtgtgcaagctctccatgcatccaattcctcagaaagatattcaatttttaaaggtactgacacctcccgacgttttaatagctgacttgtgtactcataaagtgctggaacaatgctttggtactgtcttctgatagccagtaatgcaccaatgtaaccacataatatcagcaactcatttcgagcttcagtacacgtatgcaagagtaatttttcagtacgaatatagctcagtaggtcaagaacagggtatatggtatccaaagtccagtctgagctactgatgtattctttaacaaagctaataccaataggaagggctttttcaggttcttgacttaacaagtaatattttacagtttcaaatatattgtcatctgcacgggctgtctcagctaactgcatacattcttccactgtgggtagcttacacttatcatgaaggtcatttatctcttcagtacatcctgggtagaaagcacagagttttattaaatgtagttcattatcaggaatcatcagaagaagatcagctgccaaattcctgtatccaacacatggaaagcatactgaaatcatcatgcactttctcgccagtaattctaaggcatagtgggttgctggtgctgcagactctcctagtactgtgcccacacagactgccaactccagttcatttccgcgaatcaggtatgccatagcaagctcaatattatctatggcaagatggcaacatgcggctagtactgctcgaccatcttgaaaataccattctgccagttctttactgactttgtgcaggagttcattaaagtcttccttgtagatatcatcagaatatgaagctcctttaggcacggaaacatgtaagggctgcatatttccttcacaagcagcctgtgcaacaagcagagcttctttaagctgacctcttgacatgaaaaaatggactagctttttcacatcaccaatggctatgcagtatggaatgacatcatccttatcttcctggattaattggtcagctctcctctgcattaacttcttccagtatttcacagagactcctggtgcaattgacagggctttgtcccactctccaagttcaaccataagttcacagtatctctgaatttgtcctaatctcaagtggatttcagcagcttccttcagtctttcctctttagcaggtacaccaataccaccaccaaatttagacatcttgactgttgttagttcttgagcttcagatgttctaaatttaatcagatgtttcaagtgcattattcctttgcagtagttctgaggaagtaagctatcatcctgtccttttatcacagcaaccaagttccataaattgtcactgccacctggaggagataaacattctgagaaccatcttagttttttcacttgagaattagcagttagtttttctatttcctgtctaatatctcttgacactttaccacacagtagaggaggagtgcctggttctatagcataatcagtgttcccaataatttcttcccaagatctgtctgccagaatatttatttgtacaggagtgactaaggctgttaatgaccagagtctcactgtagagtcacgggagcaagaggccatagtgaaggggcgactgggatggcaggttaaaccatatacatctgcaccgtgatcatacacagtatccacacaagttccttctcgagtgtcccatacttttatagtatagtcccagctgccagatatgagcagatatggaatctcagtattccacattaatcctctcacaggtgcagtgtgtccattaagaatattgatgcaagcatcctgagtataatcccagattcgaacggtattattgttttggctccaatcacaaccaaacactgcagctggatgtttatatttgtgtagcactttaccatcaattgttcgaataatacagaaaccatcactgctgcaggttgctattcttttagaatctttatgactccaggcaatgcagaatattccatttgttccatgctcattaaatcgttgtataattttgcccttttgaacattccaaataaaagcaccatttcgggaagttcccccagcaatacaatttaaaccacctggagcccaagaaagggaataaataacaccttcattacccggggatgtgtacactgctgttaatgtgtttatatcccagacttttatagtgccatcaaatgaagctgttgctaaaagattaggatcgtcaggtttgaatttgcagtcaaagatagtttccacatgtcccaagtctctaagaaaatcccacttcttagctcccatatcataaagtccaactccaccatccaagaaacaacacactgcatgaccaggaggaagagaaaatgcttgattctgtgttaaagttgggggtggaactgcttcgcttgttgaggatgtataatgatttttggttggagattggactgaaaacttttttcttggaggagaattaagtacatgtaagcagtgaaatcctgttttctttaatttaagattatcaataggtgttgttcttgaaacattccaaatgcgtaaaacacccacttgagaatctccagttataaacatcccaggagcactgggaacccaggctaagcactgtacagaagctgctgcactgggaagattaaatgttgttatgcaagaaagtgattcagaatctaccaggcgaattccataatgcaaattaaccactagaagataatcagtagatagtgggtcccattccaaggccgtaactggatcctcttcatctgtcccttcaagagattctggtctcaaaacatgtttctgatttttattacctggatgaaaaattgatagacttccatcaatatgaccaaacacaactttccccttttggtgtgtatgccatctgaacatacagatatcagacaagaagctatgagcatctttgtgtacaatcactccactatctggtcctgagatggtccaaatgaacagtgggcctctgtgggaaacaaatgccaccacatcctctgcattccagcaccaactaagagaagcagggatcccttttgtactgtcgagtttagcaatgactttttgttctgcaacattccaaatgatcactaaattatcagtactgccacttgcaaacagatcaggattatgtggacaccaagaaattgctgtgattgtttttttatgttcagacataattgcgtgaagtttgaattcattataacggtgatccaactgataaatatagatagccagggtcgcacaatatgcaaacctgtctccactggcagcacatacatccttgttccatggctgacatccagcagccagcaatcccacttgccttacctgggacatgtttgcctggaggaggaggcggctgcagcggcggacagcggaaggtgctgaagccggcgggcgcagctgcgaggcgagcaccaccaacgcgcggaccctccccgccctccccgcctgctcgctcagggcgcccgggggcggggcggccgggcccgcgggctccgaggggcgggaagcgtgctccgcaagccccagcgcggagccacgatggaaggcgccgcgagcccgatctccagggtctgccc

SEQ ID NO: 10836 - RNA, 5717 nt, Homo sapiens
  source 1..5717: mol_type = other RNA
ctgaatagctgggactacaggtacacaccaccacacccagctaatttttgtatttttagtagagacagggtttcaccatgttggccaggatggtctccatctaccgacctcaagatctgcccatctcggcctcctgaagtgctgggattacaggcaattttttttttttaataaaatggaatttaagcctgtaatgtctttttaaggaatcaaaagtggtcatgtgataaatatgatacatagatacataatatatattttttccagttttaagaagttttgttaagaaggttttaaaaatattttaaatgcaacaagtttaaagataataaaagccacaagtattctagttatatgagattattctttagtcaaacaaaaccatctatattataaatcttgtgaaacaacttgagtatcaaagtacttccagtatgcattaatttaataagtttcaaagtcagaattctagtccaactgaaatatctgtagtcacattatcaggcttttcatagcttcacacttttaaacaacattttaaaagttaaatcaacataatatatccaaaaattcaaccaatatctatttacaaacatttacttaaaactaattttcatcaaatcaattgtggtttttgttggtttgttttttgagacagagtttcgctctttgttgcccaggctggagtgcagtggtgcgatcttggctcactggaacctctgcctcccaggttcaagggattctcctgcctcagcttcccaagtaactgggattacaggtgcccgccaccatgcctggctaatttttgtatttttagtggagacagggttttaccatgctggccaggctggtcatgaactcctgacctcaggtgatccacctgccttggcctgccaaagtgctgagattacaggtgtgagccaccgtgcccggccaaataaattgtgttttaaataaagttaacataaattgactagagtatactgtgtaaattattgtacacattaatcaaaactaatatccatgcatgctgaatctcttaaaatagtcactttatcacctaatgcaagttttcatatatatattcgactgcattttgtgatttttacccgccaatttttttcaagcctatataacttacacctttacaatgggacagttaaacttcagataaaaaaactggtaacattttcttttttttaaaagtattttgaatgtgtatccatttattaatatttactaaacttataactgaaaacttttattaaaacagctaacgttagtggtttactatgcattttataaaggagaacgtaagtgtttgttaagttgaagatcactgtgcacaccttacatttcaacatttcaagatattcaatcattcaaatatccattaagtacttactgtatgtctagcactattctaggtgttgcacaatttaatatgtttcaatatttcaaccatatgatattttggtatcttttatgctgtgtgaaacttttatatgctttttagattattcagtcctttataatttaaatgtttcctccttcccaaacgtagctattactgtttataaaggaggcacctatttttcctttaaattatatatatatatatattttgaagttaatgactaaaattcactgctatttcccacctctcccaacctgcaatccttctcccaacctctggcacttgagcaacaaagattaaggtaatgctaacccatgaaagtttttctttaaaaaaaaaaatcaagcatggacaaaaatcttctatcagaatggattgagtcgtattccagtccctaaaggtgagaatggattcacctttgcccacatcaaagcatcattcaaggagatagcagatttcccgtcttcaaggaaaaacacagggccctggatttttaatcccgtaagacaagaaatgtgaatatcagaatgacttggaagatttgatccagtcacataatctggtccaataattcctttcagtgactcttcttttagtctctttaataaagttgcataaatcattctttgtgaatcagaagggggtgtatacggagagtcttctaatgatctgttggtggactgtgtgcaagctctccatgcatccaattcctcagaaagatattcaatttttaaaggtactgacacctcccgacgttttaatagctgacttgtgtactcataaagtgctggaacaatgctttggtactgtcttctgatagccagtaatgcaccaatgtaaccacataatatcagcaactcatttcgagcttcagtacacgtatgcaagagtaatttttcagtacgaatatagctcagtaggtcaagaacagggtatatggtatccaaagtccagtctgagctactgatgtattctttaacaaagctaataccaataggaagggctttttcaggttcttgacttaacaagtaatattttacagtttcaaatatattgtcatctgcacgggctgtctcagctaactgcatacattcttccactgtgggtagcttacacttatcatgaaggtcatttatctcttcagtacatcctgggtagaaagcacagagttttattaaatgtagttcattatcaggaatcatcagaagaagatcagctgccaaattcctgtatccaacacatggaaagcatactgaaatcatcatgcactttctcgccagtaattctaaggcatagtgggttgctggtgctgcagactctcctagtactgtgcccacacagactgccaactccagttcatttccgcgaatcaggtatgccatagcaagctcaatattatctatggcaagatggcaacatgcggctagtactgctcgaccatcttgaaaataccattctgccagttctttactgactttgtgcaggagttcattaaagtcttccttgtagatatcatcagaatatgaagctcctttaggcacggaaacatgtaagggctgcatatttccttcacaagcagcctgtgcaacaagcagagcttctttaagctgacctcttgacatgaaaaaatggactagctttttcacatcaccaatggctatgcagtatggaatgacatcatccttatcttcctggattaattggtcagctctcctctgcattaacttcttccagtatttcacagagactcctggtgcaattgacagggctttgtcccactctccaagttcaaccataagttcacagtatctctgaatttgtcctaatctcaagtggatttcagcagcttccttcagtctttcctctttagcaggtacaccaataccaccaccaaatttagacatcttgactgttgttagttcttgagcttcagatgttctaaatttaatcagatgtttcaagtgcattattcctttgcagtagttctgaggaagtaagctatcatcctgtccttttatcacagcaaccaagttccataaattgtcactgccacctggaggagataaacattctgagaaccatcttagttttttcacttgagaattagcagttagtttttctatttcctgtctaatatctcttgacactttaccacacagtagaggaggagtgcctggttctatagcataatcagtgttcccaataatttcttcccaagatctgtctgccagaatatttatttgtacaggagtgactaaggctgttaatgaccagagtctcactgtagagtcacgggagcaagaggccatagtgaaggggcgactgggatggcaggttaaaccatatacatctgcaccgtgatcatacacagtatccacacaagttccttctcgagtgtcccatacttttatagtatagtcccagctgccagatatgagcagatatggaatctcagtattccacattaatcctctcacaggtgcagtgtgtccattaagaatattgatgcaagcatcctgagtataatcccagattcgaacggtattattgttttggctccaatcacaaccaaacactgcagctggatgtttatatttgtgtagcactttaccatcaattgttcgaataatacagaaaccatcactgctgcaggttgctattcttttagaatctttatgactccaggcaatgcagaatattccatttgttccatgctcattaaatcgttgtataattttgcccttttgaacattccaaataaaagcaccatttcgggaagttcccccagcaatacaatttaaaccacctggagcccaagaaagggaataaataacaccttcattacccggggatgtgtacactgctgttaatgtgtttatatcccagacttttatagtgccatcaaatgaagctgttgctaaaagattaggatcgtcaggtttgaatttgcagtcaaagatagtttccacatgtcccaagtctctaagaaaatcccacttcttagctcccatatcataaagtccaactccaccatccaagaaacaacacactgcatgaccaggaggaagagaaaatgcttgattctgtgttaaagttgggggtggaactgcttcgcttgttgaggatgtataatgatttttggttggagattggactgaaaacttttttcttggaggagaattaagtacatgtaagcagtgaaatcctgttttctttaatttaagattatcaataggtgttgttcttgaaacattccaaatgcgtaaaacacccacttgagaatctccagttataaacatcccaggagcactgggaacccaggctaagcactgtacagaagctgctgcactgggaagattaaatgttgttatgcaagaaagtgattcagaatctaccaggcgaattccataatgcaaattaaccactagaagataatcagtagatagtgggtcccattccaaggccgtaactggatcctcttcatctgtcccttcaagagattctggtctcaaaacatgtttctgatttttattacctggatgaaaaattgatagacttccatcaatatgaccaaacacaactttccccttttggtgtgtatgccatctgaacatacagatatcagacaagaagctatgagcatctttgtgtacaatcactccactatctggtcctgagatggtccaaatgaacagtgggcctctgtgggaaacaaatgccaccacatcctctgcattccagcaccaactaagagaagcagggatcccttttgtactgtcgagtttagcaatgactttttgttctgcaacattccaaatgatcactaaattatcagtactgccacttgcaaacagatcaggattatgtggacaccaagaaattgctgtgattgtttttttatgttcagacataattgcgtgaagtttgaattcattataacggtgatccaactgataaatatagatagccagggtcgcacaatatgcaaacctgtctccactggcagcacatacatccttgttccatggctgacatccagcagccagcaatcccacttgccttacctgggacatgtttgctctttgtagtccttcataccaatcatcttgctcaaaccaatttgaaatgtaagtcatccaagccatagaatgtttctactttaatcaaggcaattggaaactcggcatcagaatagtcagcacctaaagtaacaacaatgtgtttcaaccaaacaagatttaccaaaatctcccttgtgaaatgatgttcagtacaaaaggctagaactgcacaaatattt

SEQ ID NO: 10837 - RNA, 6047 nt, Homo sapiens
  source 1..6047: mol_type = other RNA
ctgaatagctgggactacaggtacacaccaccacacccagctaatttttgtatttttagtagagacagggtttcaccatgttggccaggatggtctccatctaccgacctcaagatctgcccatctcggcctcctgaagtgctgggattacaggcaattttttttttttaataaaatggaatttaagcctgtaatgtctttttaaggaatcaaaagtggtcatgtgataaatatgatacatagatacataatatatattttttccagttttaagaagttttgttaagaaggttttaaaaatattttaaatgcaacaagtttaaagataataaaagccacaagtattctagttatatgagattattctttagtcaaacaaaaccatctatattataaatcttgtgaaacaacttgagtatcaaagtacttccagtatgcattaatttaataagtttcaaagtcagaattctagtccaactgaaatatctgtagtcacattatcaggcttttcatagcttcacacttttaaacaacattttaaaagttaaatcaacataatatatccaaaaattcaaccaatatctatttacaaacatttacttaaaactaattttcatcaaatcaattgtggtttttgttggtttgttttttgagacagagtttcgctctttgttgcccaggctggagtgcagtggtgcgatcttggctcactggaacctctgcctcccaggttcaagggattctcctgcctcagcttcccaagtaactgggattacaggtgcccgccaccatgcctggctaatttttgtatttttagtggagacagggttttaccatgctggccaggctggtcatgaactcctgacctcaggtgatccacctgccttggcctgccaaagtgctgagattacaggtgtgagccaccgtgcccggccaaataaattgtgttttaaataaagttaacataaattgactagagtatactgtgtaaattattgtacacattaatcaaaactaatatccatgcatgctgaatctcttaaaatagtcactttatcacctaatgcaagttttcatatatatattcgactgcattttgtgatttttacccgccaatttttttcaagcctatataacttacacctttacaatgggacagttaaacttcagataaaaaaactggtaacattttcttttttttaaaagtattttgaatgtgtatccatttattaatatttactaaacttataactgaaaacttttattaaaacagctaacgttagtggtttactatgcattttataaaggagaacgtaagtgtttgttaagttgaagatcactgtgcacaccttacatttcaacatttcaagatattcaatcattcaaatatccattaagtacttactgtatgtctagcactattctaggtgttgcacaatttaatatgtttcaatatttcaaccatatgatattttggtatcttttatgctgtgtgaaacttttatatgctttttagattattcagtcctttataatttaaatgtttcctccttcccaaacgtagctattactgtttataaaggaggcacctatttttcctttaaattatatatatatatatattttgaagttaatgactaaaattcactgctatttcccacctctcccaacctgcaatccttctcccaacctctggcacttgagcaacaaagattaaggtaatgctaacccatgaaagtttttctttaaaaaaaaaaatcaagcatggacaaaaatcttctatcagaatggattgagtcgtattccagtccctaaaggtgagaatggattcacctttgcccacatcaaagcatcattcaaggagatagcagatttcccgtcttcaaggaaaaacacagggccctggatttttaatcccgtaagacaagaaatgtgaatatcagaatgacttggaagatttgatccagtcacataatctggtccaataattcctttcagtgactcttcttttagtctctttaataaagttgcataaatcattctttgtgaatcagaagggggtgtatacggagagtcttctaatgatctgttggtggactgtgtgcaagctctccatgcatccaattcctcagaaagatattcaatttttaaaggtactgacacctcccgacgttttaatagctgacttgtgtactcataaagtgctggaacaatgctttggtactgtcttctgatagccagtaatgcaccaatgtaaccacataatatcagcaactcatttcgagcttcagtacacgtatgcaagagtaatttttcagtacgaatatagctcagtaggtcaagaacagggtatatggtatccaaagtccagtctgagctactgatgtattctttaacaaagctaataccaataggaagggctttttcaggttcttgacttaacaagtaatattttacagtttcaaatatattgtcatctgcacgggctgtctcagctaactgcatacattcttccactgtgggtagcttacacttatcatgaaggtcatttatctcttcagtacatcctgggtagaaagcacagagttttattaaatgtagttcattatcaggaatcatcagaagaagatcagctgccaaattcctgttaacgtaacaaaaggggacactgtatccaacacatggaaagcatactgaaatcatcatgcactttctcgccagtaattctaaggcatagtgggttgctggtgctgcagactctcctagtactgtgcccacacagactgccaactccagttcatttccgcgaatcaggtatgccatagcaagctcaatattatctatggcaagatggcaacatgcggctagtactgctcgaccatcttgaaaataccattctgccagttctttactgactttgtgcaggagttcattaaagtcttccttgtagatatcatcagaatatgaagctcctttaggcacggaaacatgtaagggctgcatatttccttcacaagcagcctgtgcaacaagcagagcttctttaagctgacctcttgacatgaaaaaatggactagctttttcacatcaccaatggctatgcagtatggaatgacatcatccttatcttcctggattaattggtcagctctcctctgcattaacttcttccagtatttcacagagactcctggtgcaattgacagggctttgtcccactctccaagttcaaccataagttcacagtatctctgaatttgtcctaatctcaagtggatttcagcagcttccttcagtctttcctctttagcaggtacaccaataccaccaccaaatttagacatcttgactgttgttagttcttgagcttcagatgttctaaatttaatcagatgtttcaagtgcattattcctttgcagtagttctgaggaagtaagctatcatcctgtccttttatcacagcaaccaagttccataaattgtcactgccacctggaggagataaacattctgagaaccatcttagttttttcacttgagaattagcagttagtttttctatttcctgtctaatatctcttgacactttaccacacagtagaggaggagtgcctggttctatagcataatcagtgttcccaataatttcttcccaagatctgtctgccagaatatttatttgtacaggagtgactaaggctgttaatgaccagagtctcactgtagagtcacgggagcaagaggccatagtgaaggggcgactgggatggcaggttaaaccatatacatctgcaccgtgatcatacacagtatccacacaagttccttctcgagtgtcccatacttttatagtatagtcccagctgccagatatgagcagatatggaatctcagtattccacattaatcctctcacaggtgcagtgtgtccattaagaatattgatgcaagcatcctgagtataatcccagattcgaacggtaccatcatcagaaccactgcaaagaattccctctctcagaggagaccatttaacatgaaacacttttgctgtatgcccactaaatactttcaatggttgatctgagctggtggctacataataaacacgaacatttgtgtcttcacagccagtggctatcatgtctttattgttttggctccaatcacaaccaaacactgcagctggatgtttatatttgtgtagcactttaccatcaattgttcgaataatacagaaaccatcactgctgcaggttgctattcttttagaatctttatgactccaggcaatgcagaatattccatttgttccatgctcattaaatcgttgtataattttgcccttttgaacattccaaataaaagcaccatttcgggaagttcccccagcaatacaatttaaaccacctggagcccaagaaagggaataaataacaccttcattacccggggatgtgtacactgctgttaatgtgtttatatcccagacttttatagtgccatcaaatgaagctgttgctaaaagattaggatcgtcaggtttgaatttgcagtcaaagatagtttccacatgtcccaagtctctaagaaaatcccacttcttagctcccatatcataaagtccaactccaccatccaagaaacaacacactgcatgaccaggaggaagagaaaatgcttgattctgtgttaaagttgggggtggaactgcttcgcttgttgaggatgtataatgatttttggttggagattggactgaaaacttttttcttggaggagaattaagtacatgtaagcagtgaaatcctgttttctttaatttaagattatcaataggtgttgttcttgaaacattccaaatgcgtaaaacacccacttgagaatctccagttataaacatcccaggagcactgggaacccaggctaagcactgtacagaagctgctgcactgggaagattaaatgttgttatgcaagaaagtgattcagaatctaccaggcgaattccataatgcaaattaaccactagaagataatcagtagatagtgggtcccattccaaggccgtaactggatcctcttcatctgtcccttcaagagattctggtctcaaaacatgtttctgatttttattacctggatgaaaaattgatagacttccatcaatatgaccaaacacaactttccccttttggtgtgtatgccatctgaacatacagatatcagacaagaagctatgagcatctttgtgtacaatcactccactatctggtcctgagatggtccaaatgaacagtgggcctctgtgggaaacaaatgccaccacatcctctgcattccagcaccaactaagagaagcagggatcccttttgtactgtcgagtttagcaatgactttttgttctgcaacattccaaatgatcactaaattatcagtactgccacttgcaaacagatcaggattatgtggacaccaagaaattgctgtgattgtttttttatgttcagacataattgcgtgaagtttgaattcattataacggtgatccaactgataaatatagatagccagggtcgcacaatatgcaaacctgtctccactggcagcacatacatccttgttccatggctgacatccagcagccagcaatcccacttgccttacctgggacatgtttgctctttgtagtccttcataccaatcatcttgctcaaaccaatttgaaatgtaagtcatccaagccatagaatgtttctactttaatcaaggcaattggaaactcggcatcagaatagtcagcacctggaggaggaggcggctgcagcggcggacagcggaaggtgctgaagccggcgggcgcagctgcgaggcgagcaccaccaacgcgcggaccctccccgccctccccgcctgctcgctcagggcgcccgggggcggggcggccgggcccgcgggctccgaggggcgggaagcgtgctccgcaagccccagcgcggagccacgatggaaggcgccgcgagcccgatctccagggtctgccc

SEQ ID NO: 10838 - RNA, 3692 nt, Homo sapiens
  source 1..3692: mol_type = other RNA
ctgaatagctgggactacaggtacacaccaccatgcccagctaatttttattttttattttgtagagatggagtctcactgtgttgcccaggctggacttgaactttcaggctcaagtaattctcccacctcagcctcccaaagtgttgggattacaggcgtgagcccttgctcctggcctagattgttttcttaatttctttttggaataatttgttagtgtatagaaatgccattggtttttctatgttgggttttgtgtcctataactttactgaattcatttattagttttgaaaatttttgatggagtctttagcattttccatataagatcatgttgtctgcaaacagacaatttaacttcttattttcctatttgcatcccttttatttctttccgttgcctaatttctctggctaggactttcagtactattgcaaccagacgtttttatagatatttgtatcagttagctgtggctaagttgtgctgtggtaataagcaatttcaaaccaatttcagtggcttgccacaacaaaaatttctttcttacatattgactatgaattgactgtgactctgccccattctgggatccacactgaagacatagttttctgtgccatgcccatctagggcagaaagaaaaagtagtggctcttacagacttatggtcaaaagtggcacatatcaatccactcacatttcactgaacaaagcaagtcaaatggccaagcatgatttcagtgtgtgggaaatagaaatcttctcatagtgtggacactgaaagaatacagcaatgggttggaatgtataattcttttttttttttttgagacagtcttgctctgtcacccaggctagagtgcagtggcgcgatctcggctcactgcaacctccacctcctgggttcaagtgattctcctatctcagcctcccgagtagctgggattacaggcatgtgccaccacacctggctaatttttgtatttttagtagagatggggtttcactatgttggccaggctggtctcaaaactcctgacctcaggtgatccaccggccttggcctccaaaagtgctgggattacaggcttgagccactgcacccggcctggaatctataattctttcacagggtagagcagaaactatttggaacaataatacaatttactgcagtatgatctcatcattcagttctaagtattctctaatttgcatcatatttttttccattggatccataaattatttagaagtgattctcttaatttctgaaagagtatctttcacttattgatttccaaggtaatgagattatggccagacagtgagatctgtatgattccaatccttgaaaattacttgagatttgctttatgcttcagtatatggacagtttgtgcaagtgatctgaatgtgcttgagaaaaacatgctattttctaattattggctaaaatgttctctgtatgtcatgtagttcaatcctattgattgtgtaattcttttttggagggttgagggatggtagcaaagaacctattggttttgtgccccacccactgattgtataattcaaatatatattattactgatatattttttgtctcattgataagctgtcaattcctgagagagagagagagagagcagcaaaagtgcttatgtgtagaaagtagtctacttgcatgcagtgtgcaaagccttatgtagaagagtctacagagagaggagagaacctcagtgaactgctggattgttaaagcagagatctgttagggagtatctaaggcagcattgtttaaaatttttaaacaaggaagattgttggtcagacgcagttactcacacctgtgatcccaacactttgggaggccaacgtgggaggatggcttgagcccaggagttcgagactagtctgggcaatatggtaagaccctgtctctccagaggaaaaaaaaaaaaagaagccaagcatggtggtgcacacctgtggtcccagctacttgggaggctgaggtgggaagatggcttgagcccagagagttgaggctgcagtgagctgtgattgtaccagtgcactccaatgtgggtgatagagctagacccccaagaatatattgacaggagtgaggctctagcatatatacagtaacagcatgaggtgaatctgattctttgcactttagttttacagtcacctgtcttggtttgtcagttatatcacaaatatctccatttccataaaaatgtgacaccatcctgactgtctgggtaccatcgtcttgaagatgataagctctagcagtattcttcttagcccattcaatatgctcttcttggttccatgtcccgacaaccacagaggttttcccactatccttgtcctcatggtattgatgtacatgtttgccatagcagaattcatatttccaccaaccgacacccccacgaaagcagtaagaaccactaagaaactcttttatgagttggtcatctgtcaatttggatatgtgggttgtcccaacagtgagcactggctgagagccaatagcaatcgacttgtggatcgctggaaatctctcttctttagttgattgcaaatcttcctctttatttctcctaaaaggcacccttagtatttcttcctgctgctccagctgcctcagggtgaggggcttaaatggagatcctggcagtgattgacaaaatatgtcattcacaggagatgctctgaacctatatttaggatgactgcacaagagtggtgtcaaaatgacaacttcatattcacaagttgtaacttcagctactgaaagaatttcatgcttagattcaggatgacatatgtacatcacagtacttgatctgggccggttctgtttcaaactacaaggtgtaccatttcccattcccacaggatagtatggtgtcatctgaccttcgatatttttagtgggaatctcatttgatttttccttttcttctgcttctcgttctttttcaaatagaaggttcttggccaacatattcccaaggtagtactcgtgaatatttattttctgaccagtttctttctcttcatggtactgccgaatgtgttttccatgacatacttcgtaagtccaataagactcaattctgtaggaacaactgctttgtttaaatagtggctccaaaagctctcttggattagggcctttataatccttttcttcttcctcatccccacttgtcacaaggggaagtatgcatttatatttttctttatgtgcagttgtcatgatgacataattatcttctttatataaaactccagttgtgggcagagagaactcggtgccgggccagttgactcggaaagggatgtcatcgctgagttgaggaagggctcggccgccgccggacgcctccaggaggccgcagaggaccagtaacaccggcccgcccgggaccagactccgtacgccgccgcctccttcctccatcctccgccgccgctttctccagccaccgccacaacctcctctgctccaggaggagaggaggaggaggaggaggtggaggaggaggcggcgggactataaagcgcccgggtatcaccggcccaaccgccgccacgtctccttccggagagcccggcaacgccgcctccgcccccttgagcctcctgtcaccgttt

SEQ ID NO: 10839 - RNA, 3530 nt, Homo sapiens
  source 1..3530: mol_type = other RNA
ctgaatagctgggactacaggtacacaccaccatgcccagctaatttttattttttattttgtagagatggagtctcactgtgttgcccaggctggacttgaactttcaggctcaagtaattctcccacctcagcctcccaaagtgttgggattacaggcgtgagcccttgctcctggcctagattgttttcttaatttctttttggaataatttgttagtgtatagaaatgccattggtttttctatgttgggttttgtgtcctataactttactgaattcatttattagttttgaaaatttttgatggagtctttagcattttccatataagatcatgttgtctgcaaacagacaatttaacttcttattttcctatttgcatcccttttatttctttccgttgcctaatttctctggctaggactttcagtactattgcaaccagacgtttttatagatatttgtatcagttagctgtggctaagttgtgctgtggtaataagcaatttcaaaccaatttcagtggcttgccacaacaaaaatttctttcttacatattgactatgaattgactgtgactctgccccattctgggatccacactgaagacatagttttctgtgccatgcccatctagggcagaaagaaaaagtagtggctcttacagacttatggtcaaaagtggcacatatcaatccactcacatttcactgaacaaagcaagtcaaatggccaagcatgatttcagtgtgtgggaaatagaaatcttctcatagtgtggacactgaaagaatacagcaatgggttggaatgtataattcttttttttttttttgagacagtcttgctctgtcacccaggctagagtgcagtggcgcgatctcggctcactgcaacctccacctcctgggttcaagtgattctcctatctcagcctcccgagtagctgggattacaggcatgtgccaccacacctggctaatttttgtatttttagtagagatggggtttcactatgttggccaggctggtctcaaaactcctgacctcaggtgatccaccggccttggcctccaaaagtgctgggattacaggcttgagccactgcacccggcctggaatctataattctttcacagggtagagcagaaactatttggaacaataatacaatttactgcagtatgatctcatcattcagttctaagtattctctaatttgcatcatatttttttccattggatccataaattatttagaagtgattctcttaatttctgaaagagtatctttcacttattgatttccaaggtaatgagattatggccagacagtgagatctgtatgattccaatccttgaaaattacttgagatttgctttatgcttcagtatatggacagtttgtgcaagtgatctgaatgtgcttgagaaaaacatgctattttctaattattggctaaaatgttctctgtatgtcatgtagttcaatcctattgattgtgtaattcttttttggagggttgagggatggtagcaaagaacctattggttttgtgccccacccactgattgtataattcaaatatatattattactgatatattttttgtctcattgataagctgtcaattcctgagagagagagagagagagcagcaaaagtgcttatgtgtagaaagtagtctacttgcatgcagtgtgcaaagccttatgtagaagagtctacagagagaggagagaacctcagtgaactgctggattgttaaagcagagatctgttagggagtatctaaggcagcattgtttaaaatttttaaacaaggaagattgttggtcagacgcagttactcacacctgtgatcccaacactttgggaggccaacgtgggaggatggcttgagcccaggagttcgagactagtctgggcaatatggtaagaccctgtctctccagaggaaaaaaaaaaaaagaagccaagcatggtggtgcacacctgtggtcccagctacttgggaggctgaggtgggaagatggcttgagcccagagagttgaggctgcagtgagctgtgattgtaccagtgcactccaatgtgggtgatagagctagacccccaagaatatattgacaggagtgaggctctagcatatatacagtaacagcatgaggtgaatctgattctttgcactttagttttacagtcacctgtcttggtttgtcagttatatcacaaatatctccatttccataaaaatgtgacaccatcctgactgtctgggtaccatcgtcttgaagatgataagctctagcagtattcttcttagcccattcaatatgctcttcttggttccatgtcccgacaaccacagaggttttcccactatccttgtcctcatggtattgatgtacatgtttgccatagcagaattcatatttccaccaaccgacaccctctttatttctcctaaaaggcacccttagtatttcttcctgctgctccagctgcctcagggtgaggggcttaaatggagatcctggcagtgattgacaaaatatgtcattcacaggagatgctctgaacctatatttaggatgactgcacaagagtggtgtcaaaatgacaacttcatattcacaagttgtaacttcagctactgaaagaatttcatgcttagattcaggatgacatatgtacatcacagtacttgatctgggccggttctgtttcaaactacaaggtgtaccatttcccattcccacaggatagtatggtgtcatctgaccttcgatatttttagtgggaatctcatttgatttttccttttcttctgcttctcgttctttttcaaatagaaggttcttggccaacatattcccaaggtagtactcgtgaatatttattttctgaccagtttctttctcttcatggtactgccgaatgtgttttccatgacatacttcgtaagtccaataagactcaattctgtaggaacaactgctttgtttaaatagtggctccaaaagctctcttggattagggcctttataatccttttcttcttcctcatccccacttgtcacaaggggaagtatgcatttatatttttctttatgtgcagttgtcatgatgacataattatcttctttatataaaactccagttgtgggcagagagaactcggtgccgggccagttgactcggaaagggatgtcatcgctgagttgaggaagggctcggccgccgccggacgcctccaggaggccgcagaggaccagtaacaccggcccgcccgggaccagactccgtacgccgccgcctccttcctccatcctccgccgccgctttctccagccaccgccacaacctcctctgctccaggaggagaggaggaggaggaggaggtggaggaggaggcggcgggactataaagcgcccgggtatcaccggcccaaccgccgccacgtctccttccggagagcccggcaacgccgcctccgcccccttgagcctcctgtcaccgttt

SEQ ID NO: 10840 - RNA, 3400 nt, Homo sapiens
  source 1..3400: mol_type = other RNA
ctgaatagctgggactacaggtacacaccaccatgtctggatacattttgtatttttggtagacaccgggtttcaccatgttgcccaggctggcctcaaactcctgggctcaagtgatctgcctgtcttggcctcccatcgtgctgggattagaggcatgagcgactgtgccaggctgactgtggacaagttttacaaataaaccaaaataaaaatattttcacttttcagctgcacatggtggaaatgtacatgtatgatgacaaagtcggagatatttattacgctgaagacatttaactttgttccatgccagccatgagtgacaacgctagagattccaaatggggaaaggatcctctacagacggctttgtttaaaatggttacaagaaacatatggcagtttttaaaatcagattccattttctctatagattccattcgccaagtgcccaggcctgcctgccaaccgtctgcaaacatgagagccaagttcaacaccttcatgatagcttctttcacaaagctgaccttttctctcagcagacaccggtcatggatggttgacagatacctatagtgaattttaatcaattgatctaaatccttggcttcctcgacttgatgttgaaactccagccctgtactgtgtagaatcctggtcatgatgtagttgtgcaagctgttcacgaaatgcatgagcttcactcttaagaggaacatgcgatgaatctgctgtcttactggttctttttgtggtccgaactgagcaactgtgtcttgttcatgtataaggccttctttaagtcgtggtttttctgcagtactaaccagttcaccaaaaagtaaaacatccagactatattttgcccactttatttgcaataagagaagaaacacttgattataaattttttgacattccaaacttataacaatgtccacgggccatgggaccttgtagctgagggtcagaccatctaagatatgaacaggcagcttcttcttagctgtgtcaacattttcaaaagatatagatagacgtgaactatcttcaggataacgctgtcctactgcttcttggagttggacattaagaaaagacacattctgccatgtttccttttctcttattttatcaaaaattgacgtgtagaagtcatacatggtatctcctccttccattaagaaaaaattcctcatagcttgcaagtattctaccaacctgtaatctttttttagagtttgcatgagatttccacagcaatctagatactgcttgtcaatatgaggatagaggcaggatctcagcgttaattcaaaagtctggcatgtcacagattccgatgatctatccacacatacatcaccaccagcaaacttctcgtgaaagtcactctgctccaaatacatccttgcaaagttaatggcaagcagtggatcatgaacatcatccagttcaagatggctttcagcaatggactgcatcttcatcaggttctccttggttgcctgttgctcagtaagaacctgtggagtggaatcttctccatgtcgaagacgggactgtacagattccagaaagagagtgtataaactttttctttctgcatctctggctcctgcctggcaggtggtgctctccgcacactgcaggttcttcagcagctgcatcgacttgccagccattatgatctgcttcaggacaggtttgaggaaggacaccatggtgtgctgcctgctggagggcccctggtcactgccggaactcgcactagcgttatcactcattttttcttcattttctgtcttttctgatacgctatataacgtgtaagttgcataccagaagtctctgtgattaactggaacatttttgtttctctggatgatgaactccctggcgccatcccacaggtgcccgtgcacgatccactcgtccaccgtctgcaggtaaggccgcaccgtttccacccagagagagaaaaggagggagacggtttgctcagaggcttctccaacattgtcatattcaagaatggccttgtacagggtgttaagcaggtgagaggcccggacgacatttcgagtatcaggtggaacttctgctactccagtactaaacactttgtgcagaaccttgagctgagacaatcgaggtgccaacttgtccaccactattgcaagagttattgtagtatcattattgatgatgcacttctcaatttctgcaagttcctctttgaaactaatgaaatatttgtacagggcccacatgaaagcctggtaggttctaaagggagcttcagttgacttcttaggaacagacccacttccaggcagcatgctctcagaactgtgtcccatgacttcatcaatgaactcctggagtcgaaacacaacctggccatatgctgctatttgttccagcacagatcgtaaacagctatgtgttaaatgagttactataatattgtttctcacagttaccttcccatctatcaactgaaatataaagagctttttcactcctgaaagtaaccatagggtttcccgaataacctgagtctcagtaaccaaaaccctgtcatctggaacatacaatggatcactgctgtacaagtgttggtcccagacagcagctaaattagagtgcaaatgtaaactatgaggaaactgggagggcctggctgtccagtactgatggaccacatgatgttccagccagcttcggtcatctggctcatctgctttccaactgatacaaggatccagttttctgttttgatcttgttcttctaacggtgtcctgtctacctgaattccagagtcctctctgcttaagggctgttgatcattttcctcttcactttcttcagaccaatttggtgtgtccatgtacggaccaatgtccatttcttcatcttccatcaagtattttccccagtcgaaatcatctttcttttccacttctttatttcttggtgtctccacataactgctgtttgaaggagagtctgacagacacagaagaagtgacagtatggaataatgtgcatctgtctttatttcctttatactgggaagtggtgcatttagaaattcctccgttaatctcttccaactagcagctttgcttagatcagaatgaatgacaaatttttcataaattccttcgattgttttttctattttgtggctgttgacatccaagaaacgatgaaatctgaagttggaccaggcgaagtttagggcgagctggaagttggggtctgcctcgtcctggaggccggcgacaccccggacgagctcccgcacgtcgcgctcctgctgcgcgtccaaccgactccacggtggcccgtgccgcgccatgttccgcgctcctgcagcgcgcgtct

SEQ ID NO: 10841 - RNA, 3397 nt, Homo sapiens
  source 1..3397: mol_type = other RNA
ctgaatagctgggactacaggtacacaccaccatgtctggatacattttgtatttttggtagacaccgggtttcaccatgttgcccaggctggcctcaaactcctgggctcaagtgatctgcctgtcttggcctcccatcgtgctgggattagaggcatgagcgactgtgccaggctgactgtggacaagttttacaaataaaccaaaataaaaatattttcacttttcagctgcacatggtggaaatgtacatgtatgatgacaaagtcggagatatttattacgctgaagacatttaactttgttccatgccagccatgagtgacaacgctagagattccaaatggggaaaggatcctctacagacggctttgtttaaaatggttacaagaaacatatggcagtttttaaaatcagattccattttctctatagattccattcgccaagtgcccaggcctgcctgccaaccgtctgcaaacatgagagccaagttcaacaccttcatgatagcttctttcacaaagctgaccttttctctcagcagacaccggtcatggatggttgacagatacctatagtgaattttaatcaattgatctaaatccttggcttcctcgacttgatgttgaaactccagccctgtactgtgtagaatcctggtcatgatgtagttgtgcaagctgttcacgaaatgcatgagcttcactcttaagaggaacatgcgatgaatctgctgtcttactggttctttttgtggtccgaactgagcaactgtgtcttgttcatgtataaggccttctttaagtcgtggtttttctgcagtactaaccagttcaccaaaaagtaaaacatccagactatattttgcccactttatttgcaataagagaagaaacacttgattataaattttttgacattccaaacttataacaatgtccacgggccatgggaccttgtagctgagggtcagaccatctaagatatgaacaggcagcttcttcttagctgtgtcaacattttcaaaagatatagatagacgtgaactatcttcaggataacgctgtcctactgcttcttggagttggacattaagaaaagacacattctgccatgtttccttttctcttattttatcaaaaattgacgtgtagaagtcatacatggtatctcctccttccattaagaaaaaattcctcatagcttgcaagtattctaccaacctgtaatctttttttagagtttgcatgagatttccacagcaatctagatactgcttgtcaatatgaggatagaggcaggatctcagcgttaattcaaaagtctggcatgtcacagattccgatgatctatccacacatacatcaccaccagcaaacttctcgtgaaagtcactctgctccaaatacatccttgcaaagttaatggcaagcagtggatcatgaacatcatccagttcaagatggctttcagcaatggactgcatcttcatcaggttctccttggttgcctgttgctcagtaagaacctgtggagtggaatcttctccatgtcgaagacgggactgtacagattccagaaagagagtgtataaactttttctttctgcatctctggctcctgcctggcaggtggtgctctccgcacactgcaggttcttcagcagctgcatcgacttgccagccattatgatctgcttcaggacaggtttgaggaaggacaccatggtgtgctgcctgctggagggcccctggtcactgccggaactcgcactagcgttatcactcattttttcttcattttctgtcttttctgatacgctatataacgtgtaagttgcataccagaagtctctgtgattaactggaacatttttgtttctctggatgatgaactccctggcgccatcccacaggtgcccgtgcacgatccactcgtccaccgtctgcaggtaaggccgcaccgtttccacccagagagagaaaaggagggagacggtttgctcagaggcttctccaacattgtcatattcaagaatggccttgtacagggtgttaagcaggtgagaggcccggacgacatttcgagtatcaggtggaacttctgctactccagtactaaacactttgtgcagaaccttgagctgagacaatcgaggtgccaacttgtccaccactattgcaagagttattgtagtatcattattgatgatgcacttctcaatttctgcaagttcctctttgaaactaatgaaatatttgtacagggcccacatgaaagcctggtaggttctaaagggagcttcagttgacttcttaggaacagacccacttccaggcagcatgctctcagaactgtgtcccatgacttcatcaatgaactcctggagtcgaaacacaacctggccatatgctgctatttgttccagcacagatcgtaaacagctatgtgttaaatgagttactataatattgtttctcacagttaccttcccatctatcaactgaaatataaagagctttttcactcctgaaagtaaccatagggtttcccgaataacctgagtctcagtaaccaaaaccctgtcatctggaacatacaatggatcactgctgtacaagtgttggtcccagacagcagctaaattagagtgcaaatgtaaactatgaggaaactgggagggcctggctgtccagtactgatggaccacatgatgttccagccagcttcggtcatctggctcatctttccaactgatacaaggatccagttttctgttttgatcttgttcttctaacggtgtcctgtctacctgaattccagagtcctctctgcttaagggctgttgatcattttcctcttcactttcttcagaccaatttggtgtgtccatgtacggaccaatgtccatttcttcatcttccatcaagtattttccccagtcgaaatcatctttcttttccacttctttatttcttggtgtctccacataactgctgtttgaaggagagtctgacagacacagaagaagtgacagtatggaataatgtgcatctgtctttatttcctttatactgggaagtggtgcatttagaaattcctccgttaatctcttccaactagcagctttgcttagatcagaatgaatgacaaatttttcataaattccttcgattgttttttctattttgtggctgttgacatccaagaaacgatgaaatctgaagttggaccaggcgaagtttagggcgagctggaagttggggtctgcctcgtcctggaggccggcgacaccccggacgagctcccgcacgtcgcgctcctgctgcgcgtccaaccgactccacggtggcccgtgccgcgccatgttccgcgctcctgcagcgcgcgtct

SEQ ID NO: 10842 - RNA, 1412 nt, Homo sapiens
  source 1..1412: mol_type = other RNA
ctgaatagctgggactacaggtacacaccactaaatccagataattttttattattaattttttggtagggatggggtctcggtatgttgcccaggctagtctccaattcctaggctcaagtgatcctcctgctttggcctcccaaagtgctgggattgtaggcatgagcctatcttagagaagtcttaagcctatgcttcccaaggcctggctgattgcttggaacatagtaagtattctgtatgtgtaggtgctattatttgttcaaccaatgttgagcaaatgaaggaaactggcaccattggcaggaaaagtctgcccctctgcagatattaggagatgatgagattcagggtgggatggtgaggacaatgaagtgagtgagtagagcaccgtggcctgcagtgtggagagggtagggggcaagaagagtgaggaggaggaggaccaccagtgccatccctagccccagctctagcaatggcggcctgactcagggctgctggccacacagaaggagacccccggcagcaaccatctctaggattctgagatgcaagtctatcatcagcatccaaaaattatgattaaaaatttagtcaattacttattgcatgcctgtgccaaaatatctcccgtaacccatatatgtgtgtgtatgtatacatatgcacctactatgtacccacaaaaattaaaaatttttaaatgtttaatcacaagtctgtagcatgacatcattagtagagtcgagtctgctgacattacaatctattgatctccccagagttaccaaaagtagttcacaatagttaggcttccttctgtccatagttcagggcatattcaaagtctctaaagctgacgtgaccatctgaatctcgatctacttccctgaatacctcaagaacagtcctttccggtaatttgggagccacctgcctaaatgcttttttgaaatcttccaaagttaaaaatccacgatagtaggtgtcaaaggctgtgaagatgtgtcttacttcgttccgatatcgttgagcttccttctttttcctgacaatatttaaaaacccctcgagtaatataccagaagtatttggatttattgaagacatcacagaatccacttctatcttggagggcttgtacccaaacagcattacaacagcagttttaaagtcctctctgctgagatatcctttgtgatcttcatcacatgctttaaataccattaatagactatatagagagaaaggagatggaacttggaggtagccgtagtcctggacggggagccaggagccctgcagctccaggatcagtcattaaccacgaccctttggacaggcagcccaggtcttatctgcacacccggcagagtgagacccagacacgggagaggaagcgagag

SEQ ID NO: 10843 - RNA, 1275 nt, Homo sapiens
  source 1..1275: mol_type = other RNA
ctgaatagctgggactacaggtacacaccactaaatccagataattttttattattaattttttggtagggatggggtctcggtatgttgcccaggctagtctccaattcctaggctcaagtgatcctcctgctttggcctcccaaagtgctgggattgtaggcatgagcctatcttagagaagtcttaagcctatgcttcccaaggcctggctgattgcttggaacatagtaagtattctgtatgtgtaggtgctattatttgttcaaccaatgttgagcaaatgaaggaaactggcaccattggcaggaaaagtctgcccctctgcagatattaggagatgatgagattcagggtgggatggtgaggacaatgaagtgagtgagtagagcaccgtggcctgcagtgtggagagggtagggggcaagaagagtgaggaggaggaggaccaccagtgccatccctagccccagctctagcaatggcggcctgactcagggctgctggccacacagaaggagacccccggcagcaaccatctctaggattctgagatgcaagtctatcatcagcatccaaaaattatgattaaaaatttagtcaattacttattgcatgcctgtgccaaaatatctcccgtaacccatatatgtgtgtgtatgtatacatatgcacctactatgtacccacaaaaattaaaaatttttaaatgtttaatcacaagtctgtagcatgacatcattagtagagtcgagtctgctgacattacaatctattgatctccccagagttaccaaaagtagttcacaatagttaggcttccttctgtccatagttcagggcatattcaaagtctctaaagctgacgtgaccatctgaatctcgatctacttccctgaatacctcaagaacagtcctttccggtaatttgggagccacctgcctaaatgcttttttgaaatcttccaaagttaaaaatccacgatagtaggtgtcaaaggctgtgaagatgtgtcttacttcgttccgatatcgttgagcttccttctttttcctgacaatatttaaaaacccctcgagtaatataccagaagtatttggatttattgaagacatcacagaatccacttctatcttggagggcttgtacccaaacagcattacaacagcagttttaaagtcctctctgctgagatatcctttgtgatcttcatcacatgctttaaataccgcggccacgcccaccgcggctcaggaagccgaacttcaccgcgc

SEQ ID NO: 10844 - RNA, 1375 nt, Homo sapiens
  source 1..1375: mol_type = other RNA
ctgaatagctgggactacaggtacacaccactaaatccagataattttttattattaattttttggtagggatggggtctcggtatgttgcccaggctagtctccaattcctaggctcaagtgatcctcctgctttggcctcccaaagtgctgggattgtaggcatgagcctatcttagagaagtcttaagcctatgcttcccaaggcctggctgattgcttggaacatagtaagtattctgtatgtgtaggtgctattatttgttcaaccaatgttgagcaaatgaaggaaactggcaccattggcaggaaaagtctgcccctctgcagatattaggagatgatgagattcagggtgggatggtgaggacaatgaagtgagtgagtagagcaccgtggcctgcagtgtggagagggtagggggcaagaagagtgaggaggaggaggaccaccagtgccatccctagccccagctctagcaatggcggcctgactcagggctgctggccacacagaaggagacccccggcagcaaccatctctaggattctgagatgcaagtctatcatcagcatccaaaaattatgattaaaaatttagtcaattacttattgcatgcctgtgccaaaatatctcccgtaacccatatatgtgtgtgtatgtatacatatgcacctactatgtacccacaaaaattaaaaatttttaaatgtttaatcacaagtctgtagcatgacatcattagtagagtcgagtctgctgacattacaatctattgatctccccagagttaccaaaagtagttcacaatagttaggcttccttctgtccatagttcagggcatattcaaagtctctaaagctgacgtgaccatctgaatctcgatctacttccctgaatacctcaagaacagtcctttccggtaatttgggagccacctgcctaaatgcttttttgaaatcttccaaagttaaaaatccacgatagtaggtgtcaaaggctgtgaagatgtgtcttacttcgttccgatatcgttgagcttccttctttttcctgacaatatttaaaaacccctcgagtaatataccagaagtatttggatttattgaagacatcacagaatccacttctatcttggagggcttgtacccaaacagcattacaacagcagttttaaagtcctctctgctgagatatcctttgtgatcttcatcacatgctttaaatacttccacccacttcctgtgttccgagggactggcttcccacgtccgcgacctggctctggcctcggagaagaacatcgcgactacaacaaccgagccccagcaacccaaccagctaccaccgctttcccagcctggctggcagcct

SEQ ID NO: 10845 - RNA, 3021 nt, Homo sapiens
  source 1..3021: mol_type = other RNA
ctgaatagctgggactacaggtacacgccacatcaggctaatttttttttaaatttttatgttttatagagtcgaggtctcactatgctgcccaggctggtctcaagctcctggcctctcaagtgatcctcccaacttatcctccagagtagctgggattataagcacagaccaccacacctagctgattcttttattctgctcataataaataaaaggctgtgataagaaaagccacagggctggaaagagtccacaaatcctccgttttctgaggtgtctattttctgccattcaggaatgtggtgcctacaaaactcaggaaaggaaggtaataattaaaaaagctcaagccacaaatagtatagctagacacacatcttactagccaggagtttcaccagcaagcggtctctattctgttttaaaagaacatagcttctttctcttgctgaggtttatatggccacagtgtaggcttcttggagttccctgattttctgctcaggtcacatatactattaaaaatcacacattcattttcaaagtattaaaatataatcaaatagattcaacactaaaattaagctgaacataatttattctttttcttggacatgatgtgagaaataaaacatcctggcctgggagtcagaagattaggttttcttgatctcaaggctgagtggtctcgaccaagttacttaacctttctaggcctccttttcctctgacgaaaaacaagggagttgcactggataagttttaaagtcccttttcaaatttcattgaaacactaagtcatgatcttgaacagtgcctcttgactatgaagatcaactaccattagagtgtaaaattaattctagtgtttgcaattttctgatgcttatattatgttaatgggagttttctatacttccaggagccaatcattagaatttggctaataaaaacataactgagattttttttttttacactgtacataaagtttactttggcattcacagggatgatctggagagagctttttgttatacatgttcttattttattctcttattgttgaaatcctattctgttctcaagtgagtggcaaaagagtagcataaaagagagataacttggttaaggtatttcttactgagataaaagaataatagaagtatttttattctttaatttttttacattttaattttttcaattttcagaacttaattttttgaactattgctaacacttaaaagcaaggatttttcataggtttaccactactggtaaagagttatgattacttccaaaatattaatatcgtgccaaagaaaacagagtttgttaccatttttatgtatatagcaatgtattttactagttatcttgataattttcagaaatgggacaaaaatagaagactcatgattctgcttttactatttcaaaccagatgttaagcatgttgaattcaaatttagaaaaggactctgtggagtgccagctacaactttgggagtaggataaataatttcttcaacagttatatatgtacctaataagaagccaacaactccagtgaatgctatagaaatatttttcaggaccatccatatattataatgttccttcgaaaatgtaagaatttcaaccaaaggtggcaggattagggccaatgtgctgctgctcacagctccaacgaaggaaatcacaatgtctaaacgaggaataagaattgctccggcacaagtaatactaaccaagaaggatcttatcccaaattcacagatttgcttccatttagtatgaaatttggatgtgatcccagggataatgatctcatacatcttggggaagatttaaagttatgctgcctttgatttcatcatggaaacacatatatcctaaagtagctaatgttacatacaaagttgtaacaatccccatgccaatattcaacgcttgagggaaacgctttgattctttcatttggttttccagtggaaggaccactcctatgccttcaaaagcaaatacagcagtaccaaaaaagagtgggtatttcttccaaccagccactattggaaggttgtggggatctggcatgttcctgacaacatactggtaaattatcacaagactgacagccatggaaacgttggcaaggaatgaaagtacaaatagattctttagttcacgaatgaagaccaaaagaattataaatggaagaaagcaaagcatatatatccttaggtcaacacttcttctctcacaagggtttgatgaattggtactatttgaaataaacactttactctccaggaatccttcatgaacttgtttcacattttcagctaagaagacaatataaacactacagaatcccagctgtgttatcaccagaaaaaagtcaaccacactccgcccccatgctgcttgcttctgaagacaactccaaggactcacttccatagcaaagctcacagtgtcactataacctaatgttgactttttaaacctcagacatagaaagtgactgcaacgtaccaatatgtgcatacagtgaacagaaataattcctataaacacaaggctgattggtccaagcactatgcctgcattttttattgccaatggaagtcctaaaaggccagttccaatatttcctttaagaaggtgcataagagtttgtacaaatgaaatgccctcttgatcatcaagttggtaatgcttctgaacaggcagaagctcttgctcatgttcttcatctgatgtcccatcaaaattctgctcatttatcaagggcctcattacatccatatctagctcctcgcgcctcgccgccccggcagccgccggcgtcgccgccgcttccatctctcgcgggtctccaggacgccgccgcccgagtgctcactctcccgccgctgcgtggccggcgtcaggcccaggcctacctcccctgcccggagggacccgcgcctggtgcccgcctccctgccccggcgctccccaaccgcgcgg

SEQ ID NO: 10846 - RNA, 3102 nt, Homo sapiens
  source 1..3102: mol_type = other RNA
ctgaatagctgggactacaggtacacgccacatcaggctaatttttttttaaatttttatgttttatagagtcgaggtctcactatgctgcccaggctggtctcaagctcctggcctctcaagtgatcctcccaacttatcctccagagtagctgggattataagcacagaccaccacacctagctgattcttttattctgctcataataaataaaaggctgtgataagaaaagccacagggctggaaagagtccacaaatcctccgttttctgaggtgtctattttctgccattcaggaatgtggtgcctacaaaactcaggaaaggaaggtaataattaaaaaagctcaagccacaaatagtatagctagacacacatcttactagccaggagtttcaccagcaagcggtctctattctgttttaaaagaacatagcttctttctcttgctgaggtttatatggccacagtgtaggcttcttggagttccctgattttctgctcaggtcacatatactattaaaaatcacacattcattttcaaagtattaaaatataatcaaatagattcaacactaaaattaagctgaacataatttattctttttcttggacatgatgtgagaaataaaacatcctggcctgggagtcagaagattaggttttcttgatctcaaggctgagtggtctcgaccaagttacttaacctttctaggcctccttttcctctgacgaaaaacaagggagttgcactggataagttttaaagtcccttttcaaatttcattgaaacactaagtcatgatcttgaacagtgcctcttgactatgaagatcaactaccattagagtgtaaaattaattctagtgtttgcaattttctgatgcttatattatgttaatgggagttttctatacttccaggagccaatcattagaatttggctaataaaaacataactgagattttttttttttacactgtacataaagtttactttggcattcacagggatgatctggagagagctttttgttatacatgttcttattttattctcttattgttgaaatcctattctgttctcaagtgagtggcaaaagagtagcataaaagagagataacttggttaaggtatttcttactgagataaaagaataatagaagtatttttattctttaatttttttacattttaattttttcaattttcagaacttaattttttgaactattgctaacacttaaaagcaaggatttttcataggtttaccactactggtaaagagttatgattacttccaaaatattaatatcgtgccaaagaaaacagagtttgttaccatttttatgtatatagcaatgtattttactagttatcttgataattttcagaaatgggacaaaaatagaagactcatgattctgcttttactatttcaaaccagatgttaagcatgttgaattcaaatttagaaaaggactctgtggagtgccagctacaactttgggagtaggataaataatttcttcaacagttatatatgtacctaataagaagccaacaactccagtgaatgctatagaaatatttttcaggaccatccatatattataatgttccttcgaaaatgtaagaatttcaaccaaaggtggcaggattagggccaatgtgctgctgctcacagctccaacgaaggaaatcacaatgtctaaacgaggaataagaattgctccggcacaagtaatactaaccaagaaggatcttatcccaaattcacagatttgcttccatttagtatgaaatttggatgtgatcccagggataatgatctctgctggaacatagaactgaattgaatatgtcacaaaaatgccaaaggaatatagaattttcactgattgatataaccatacatcttggggaagatttaaagttatgctgcctttgatttcatcatggaaacacatatatcctaaagtagctaatgttacatacaaagttgtaacaatccccatgccaatattcaacgcttgagggaaacgctttgattctttcatttggttttccagtggaaggaccactcctatgccttcaaaagcaaatacagcagtaccaaaaaagagtgggtatttcttccaaccagccactattggaaggttgtggggatctggcatgttcctgacaacatactggtaaattatcacaagactgacagccatggaaacgttggcaaggaatgaaagtacaaatagattctttagttcacgaatgaagaccaaaagaattataaatggaagaaagcaaagcatatatatccttaggtcaacacttcttctctcacaagggtttgatgaattggtactatttgaaataaacactttactctccaggaatccttcatgaacttgtttcacattttcagctaagaagacaatataaacactacagaatcccagctgtgttatcaccagaaaaaagtcaaccacactccgcccccatgctgcttgcttctgaagacaactccaaggactcacttccatagcaaagctcacagtgtcactataacctaatgttgactttttaaaccaatatgtgcatacagtgaacagaaataattcctataaacacaaggctgattggtccaagcactatgcctgcattttttattgccaatggaagtcctaaaaggccagttccaatatttcctttaagaaggtgcataagagtttgtacaaatgaaatgccctcttgatcatcaagttggtaatgcttctgaacaggcagaagctcttgctcatgttcttcatctgatgtcccatcaaaattctgctcatttatcaagggcctcattacatccatatttttttattttggacagcgggaaaccgtaaacaaacacgccctgtcgccaagaaacaagatgggaggaaagcagcaaaaaacaaacaaactttgccaagtgagcaagctacaggtatctcctgttcattctggtcagcacgacctgttcgaaactctgggataacaaggagtaaaatgaggattcatctggagattccgaatggggctgcagcatttgaaaagcagaacaatgat

SEQ ID NO: 10847 - RNA, 3110 nt, Homo sapiens
  source 1..3110: mol_type = other RNA
ctgaatagctgggactacaggtacacgccacatcaggctaatttttttttaaatttttatgttttatagagtcgaggtctcactatgctgcccaggctggtctcaagctcctggcctctcaagtgatcctcccaacttatcctccagagtagctgggattataagcacagaccaccacacctagctgattcttttattctgctcataataaataaaaggctgtgataagaaaagccacagggctggaaagagtccacaaatcctccgttttctgaggtgtctattttctgccattcaggaatgtggtgcctacaaaactcaggaaaggaaggtaataattaaaaaagctcaagccacaaatagtatagctagacacacatcttactagccaggagtttcaccagcaagcggtctctattctgttttaaaagaacatagcttctttctcttgctgaggtttatatggccacagtgtaggcttcttggagttccctgattttctgctcaggtcacatatactattaaaaatcacacattcattttcaaagtattaaaatataatcaaatagattcaacactaaaattaagctgaacataatttattctttttcttggacatgatgtgagaaataaaacatcctggcctgggagtcagaagattaggttttcttgatctcaaggctgagtggtctcgaccaagttacttaacctttctaggcctccttttcctctgacgaaaaacaagggagttgcactggataagttttaaagtcccttttcaaatttcattgaaacactaagtcatgatcttgaacagtgcctcttgactatgaagatcaactaccattagagtgtaaaattaattctagtgtttgcaattttctgatgcttatattatgttaatgggagttttctatacttccaggagccaatcattagaatttggctaataaaaacataactgagattttttttttttacactgtacataaagtttactttggcattcacagggatgatctggagagagctttttgttatacatgttcttattttattctcttattgttgaaatcctattctgttctcaagtgagtggcaaaagagtagcataaaagagagataacttggttaaggtatttcttactgagataaaagaataatagaagtatttttattctttaatttttttacattttaattttttcaattttcagaacttaattttttgaactattgctaacacttaaaagcaaggatttttcataggtttaccactactggtaaagagttatgattacttccaaaatattaatatcgtgccaaagaaaacagagtttgttaccatttttatgtatatagcaatgtattttactagttatcttgataattttcagaaatgggacaaaaatagaagactcatgattctgcttttactatttcaaaccagatgttaagcatgttgaattcaaatttagaaaaggactctgtggagtgccagctacaactttgggagtaggataaataatttcttcaacagttatatatgtacctaataagaagccaacaactccagtgaatgctatagaaatatttttcaggaccatccatatattataatgttccttcgaaaatgtaagaatttcaaccaaaggtggcaggattagggccaatgtgctgctgctcacagctccaacgaaggaaatcacaatgtctaaacgaggaataagaattgctccggcacaagtaatactaaccaagaaggatcttatcccaaattcacagatttgcttccatttagtatgaaatttggatgtgatcccagggataatgatctctgctggaacatagaactgaattgaatatgtcacaaaaatgccaaaggaatatagaattttcactgattgatataaccatacatcttggggaagatttaaagttatgctgcctttgatttcatcatggaaacacatatatcctaaagtagctaatgttacatacaaagttgtaacaatccccatgccaatattcaacgcttgagggaaacgctttgattctttcatttggttttccagtggaaggaccactcctatgccttcaaaagcaaatacagcagtaccaaaaaagagtgggtatttcttccaaccagccactattggaaggttgtggggatctggcatgttcctgacaacatactggtaaattatcacaagactgacagccatggaaacgttggcaaggaatgaaagtacaaatagattctttagttcacgaatgaagaccaaaagaattataaatggaagaaagcaaagcatatatatccttaggtcaacacttcttctctcacaagggtttgatgaattggtactatttgaaataaacactttactctccaggaatccttcatgaacttgtttcacattttcagctaagaagacaatataaacactacagaatcccagctgtgttatcaccagaaaaaagtcaaccacactccgcccccatgctgcttgcttctgaagacaactccaaggactcacttccatagcaaagctcacagtgtcactataacctaatgttgactttttaaacctcagacatagaaagtgactgcaacgtaccaatatgtgcatacagtgaacagaaataattcctataaacacaaggctgattggtccaagcactatgcctgcattttttattgccaatggaagtcctaaaaggccagttccaatatttcctttaagaaggtgcataagagtttgtacaaatgaaatgccctcttgatcatcaagttggtaatgcttctgaacaggcagaagctcttgctcatgttcttcatctgatgtcccatcaaaattctgctcatttatcaagggcctcattacatccatatctagctcctcgcgcctcgccgccccggcagccgccggcgtcgccgccgcttccatctctcgcgggtctccaggacgccgccgcccgagtgctcactctcccgccgctgcgtggccggcgtcaggcccaggcctacctcccctgcccggagggacccgcgcctggtgcccgcctccctgccccggcgctccccaaccgcgcggcgaggagcatgc

SEQ ID NO: 10848 - RNA, 1454 nt, Homo sapiens
  source 1..1454: mol_type = other RNA
ctgaatagctgggactacaggtacacgccgccatgcctggctcttgccttggttttgacgattttgacagttgaggaggactggcccgatacatcgtaggatgcccgctactggggtttgtctgacacttttctcatgattagactgggattgtgggtctggggaggaagatcacagaggtaaagtgccctgatcagcacatccaatggagggcagctgctgtcaacatgaggcatcccttgtgatgctggcgttgcccatctggctgaggtcgtgctgattgggtctctccactgtgaagtttctcttcctccccactcgctgcagtgcactctttggtgcacatatttgcagttgctttgcagcctggtgttacggatgccactcggctccctgattgtgtagtcagcagtgttaagtgttccttcctgttggcgcacatcttgtctgttgctggtgcctgctacggagtcctccgaggggcaccccacactttccctgggatcacgtgtccaggctgctcccaggtacgcaccccacagactctgctgcagagaagggggcccatttgtggacttccctggacatgcaaccaaggagcgaactgctgatcatgggtgtctgtactccagttttgaccccattttttcaggctgccctccagaaagcctgtgcgtccccatcaatcatcccacttcctgagatgtgccaagtggaggggcgtgccgcgcttgcttgccggctgttctgcacacgggcgctaagggttctgctttctctgagtcactgagctacacccaaaaccagcatcccatcctgtgggctgtaggctcaagtgggtcattgcttggcttgggcacaatatttagaaaagttttgagccaacatgtcaacactgaggaatttcacgtgcccttttaggttttgggctgctctggaaaccccaaactgcttctttcttatggttcccaaggtaaatctgttcttctcaacgtttttcatttggaagaccccgttgccccacagcaccttatggcttctgcaaaatagactgggtccactgcaaagccctgtctccaggcagagcttttcccgccaagggctgggcagcctggctggaggcagtgagcacccatcgcaggaggtatcagagcggccccagcaggtcccgggtgtgggatggggccactgacgttcccctcgtttagcttccatagctttgtgagacaggcattctcctcgcctgccgctctgcaagctggtgggacagaagcaccttccagctttgtggatgagttctgacgcagctgcggggcaacagtgccccctcgtggctgcagccccagcctggccgctctgcctgcaactcggggcctttgcacttgccggtccctctgcctggcacatgctggcttcagtgttcataaagctccctccctcccgtcactcaggtc

SEQ ID NO: 10849 - RNA, 4249 nt, Homo sapiens
  source 1..4249: mol_type = other RNA
ctgaatagctgggactacaggtacagacgtgcaccaccatgcccagctaattaaaaaaaaatttttttttgtagagatggggtctatgttgcccaggctgtcagatttgttttgtttgaaaaaaaaattttagtcttacaaatcacaatgttaaggctcactgacagattatgagacaagcctgcaagcacttttaaggcttctaaggtaatagtaagagtattaattgtaaaacactataactcccttttacatttccaagatttaagaagagatagaatagatggagattaaattcaatgaaaacacagataagagtttaactcaaagaaaagttgtagtgatgagtttcgattctaagtttgctgtcccacaactaaagacggaatgatttaaaaaaaaaaacggcaaaacttcattttataaatggaattttaaaaatttctatttgtaatgcccacatatggtaaagatgagctatttacgtttaagaaacaactgaatcaacaagaaagtcaatacagggtttttacactttttagaaaaatgtaagtgaaagaccactctgattttctcctaaaactcaagtttcttcaagtatccttggggacgtgaaaaggaattcatgccttttctgactcaattattttagtattttcccattaagcaccagaaaagtcaatctacatgagttgtgctcccaaactgcagttactattttgtataggagaaaatggtgctttttgccaaaccacagccttattcctatcagcattgaaaaaaataaattatatatatagtattatatagacctccactgtactacatatatatatatactctctctatatatgtactatatataatatatatatatatatatatatatagacctagaggatagcactggcattcatttcactctcctatgaagtaggtattatcattctcattttacagatgaggaaaccaaggcacccaaccaaaggcatatagtaggaactggaagagctgggattaaaaacccaggaagtctggctccaaactttatattcttattcactatatagtaaaccatccatcttgtaaccctaacactcatctgtaactaatgtgttgtttcccaccagagcagtagttcttcaccagggtgattttgccctccaagttcacctcccttgtcccccaacaatccaactggggaacatctggcaatgtctggaaacatttttggttgccacaacttgggggctggggtggtgtgactggcatctagtgggcagatattaaaattcctataatgcacaggagagtcgccagaatacattatcaaacataaaacatcaatagtgctgaggctgagaaactcttcaatagaatataaattctaggagggcagcattttatagttgatcttggttgctgctacatccttaggcctagaacaatttttatacttaagtacttaatttgtccaatgaatgaatatttagctgtttgagcctagaactgggcctggtacatagctggtaggcagcaaacatttattaaaagtaattattgaataatggcggtatcaatggatgtaacaggacatagtaaattgaagtaattttagtgtttcacagtcccagttttttgggcttaatttttttcccaaatgattataaataaaaccagttctgccaaaacaagtcccttttgtaaagaatcagactttttcttaacatgaaagcctttaaaaatgtatcattcaaacagcgtgtatttaggggattagcagatacccctctattagatattatcactgattaattgctccagtagctggcaaatactttcaaaaagttttttaagagctttacaatttttaaaaagttttaaaataattctataagaattcagttcttacagaattcaattatagcatatttaagaaaaatatcgattctctaagtgcttaatccacatcactcaaagatttttataaccacaatattctaacttcaatcctgtattttaaaaaatccatagtgtaacatccatgaaagtatgttaaatcgttcctcttttacctacctcatcaaatagctactgaacattacccaaaggcatttattcgtaagtaatactgcttgatttacaaaattatttctcaaggaaaagttcaaaaggtggttatgtggatattcaaacaataccagaaaactcgctacttccttattcctgtaattaatgagtctggcttgcccagatgttaaattatgaaaccatgctgtgtaaaatgcacctattacaattaaaaccagggtaaacccgtatttatttactagcactgttaaaacattacacaaaacacattcaagtggcaagtaattataatgcaagcccttgcatggcaatccaaatttattgaactactgatgctaagttatacaaaattgcaccactttaattaaggcttttagtttacatttggccacctcaaagtagttgtaacattaggttggtcaatttaaatactgtggctccctgttggatagacacacaatctttacatccaaacattaatgcatacaaagcaacaaggcattgttaaataaaacagcaatagttactgcaaattaggccttgtgaccaattacatatgattaaaattacttcccacattcacatccacagtactcgtccaccatttaacatctcaaccaaaacgttacacatgtgaaacaatcactaacaggcaaaaatactaaacctgtatatttggtattgcaaatacacttatgcatgagcaagcaagggattcacagtgagaatctacagctgcagaagcctgaaaatgatttacaaaaattgttaaatcattaaaaaattgtttgaaaatatacacttcttgttgtagacccccactgtacacacgactataaacattgttccctatgtaaacaaaaaaaggaaacatataataagagatttgaaaagtctggacatttccttcccaacagatattaaaggcaacgtctttaatctaagacattatactgaaaggactatcatgttttaaagacaagatcaccgtctccacaggttttttaaaaattaaaaaaactatatagctgtgttaatcaaagcgcttattttgtacaataataatgaccttgaatttcttaaaaaaaattacaataagctacaagtatcaaagaagcgaagttatctggagtagtctatataggagctctttggactttcttttattatgctaaaatagtggtgcttttaggatttacattattgtactctccaatacaaagtatggggcatgttaaagtatacagtacaccattttcatacatgtacaacattggtggatgaagaatgtctcttagcagtaatactggatgtagcctctggttttaccagctgcaaactctaggactattatataagtaaaaatctctcttgtgatactggaaagtgattagaatgtgcaaactgatatagtagctttcatccgcctcttaaagggtaccaccacaggaaagtccatttaagatgttggtaggtttaacaaagttggaatgctggcactgttgaattgggcaacagttcttcagacctggctcagagctacaatgcatttagtatattaaagcagctgacatgatgactttttgcgagccttcccaggcactggagtttttctgttaatttgccgcactaggtcataaaagatctcattaacatttatttttgattttgcagaagattctaagaatgcacagttgttccattgtcttgctagattttgaccttgttccttccctacaactctttcatcttccaagtcacacttattaccaacaagaatcattggaacatcatcagtgtctttaactcgaagaatctgttctctcaggtcttgtaaatcgttaaatgtggactgtgctgtgatggaataaactaatgcaaatccttgtccatttttcatgtataaatccctcattgctgtaaattgctccaaagcagactttccaacgcctcctgagccaagaacgactagcttatactcacgcatgatgcaagcttgtcaaaacctagtacctctcacgctgtcaccgggtccctgcagccagcgtcgccccgcgctccccccgggtcgctactctaggcgccacggcggtcctgccgctgccgcgccgctccggctggtttacacgcctgaatctgggcgaggtttggcgatgtc

SEQ ID NO: 10850 - RNA, 4258 nt, Homo sapiens
  source 1..4258: mol_type = other RNA
ctgaatagctgggactacaggtacagacgtgcaccaccatgcccagctaattaaaaaaaaatttttttttgtagagatggggtctatgttgcccaggctgtcagatttgttttgtttgaaaaaaaaattttagtcttacaaatcacaatgttaaggctcactgacagattatgagacaagcctgcaagcacttttaaggcttctaaggtaatagtaagagtattaattgtaaaacactataactcccttttacatttccaagatttaagaagagatagaatagatggagattaaattcaatgaaaacacagataagagtttaactcaaagaaaagttgtagtgatgagtttcgattctaagtttgctgtcccacaactaaagacggaatgatttaaaaaaaaaaacggcaaaacttcattttataaatggaattttaaaaatttctatttgtaatgcccacatatggtaaagatgagctatttacgtttaagaaacaactgaatcaacaagaaagtcaatacagggtttttacactttttagaaaaatgtaagtgaaagaccactctgattttctcctaaaactcaagtttcttcaagtatccttggggacgtgaaaaggaattcatgccttttctgactcaattattttagtattttcccattaagcaccagaaaagtcaatctacatgagttgtgctcccaaactgcagttactattttgtataggagaaaatggtgctttttgccaaaccacagccttattcctatcagcattgaaaaaaataaattatatatatagtattatatagacctccactgtactacatatatatatatactctctctatatatgtactatatataatatatatatatatatatatatatagacctagaggatagcactggcattcatttcactctcctatgaagtaggtattatcattctcattttacagatgaggaaaccaaggcacccaaccaaaggcatatagtaggaactggaagagctgggattaaaaacccaggaagtctggctccaaactttatattcttattcactatatagtaaaccatccatcttgtaaccctaacactcatctgtaactaatgtgttgtttcccaccagagcagtagttcttcaccagggtgattttgccctccaagttcacctcccttgtcccccaacaatccaactggggaacatctggcaatgtctggaaacatttttggttgccacaacttgggggctggggtggtgtgactggcatctagtgggcagatattaaaattcctataatgcacaggagagtcgccagaatacattatcaaacataaaacatcaatagtgctgaggctgagaaactcttcaatagaatataaattctaggagggcagcattttatagttgatcttggttgctgctacatccttaggcctagaacaatttttatacttaagtacttaatttgtccaatgaatgaatatttagctgtttgagcctagaactgggcctggtacatagctggtaggcagcaaacatttattaaaagtaattattgaataatggcggtatcaatggatgtaacaggacatagtaaattgaagtaattttagtgtttcacagtcccagttttttgggcttaatttttttcccaaatgattataaataaaaccagttctgccaaaacaagtcccttttgtaaagaatcagactttttcttaacatgaaagcctttaaaaatgtatcattcaaacagcgtgtatttaggggattagcagatacccctctattagatattatcactgattaattgctccagtagctggcaaatactttcaaaaagttttttaagagctttacaatttttaaaaagttttaaaataattctataagaattcagttcttacagaattcaattatagcatatttaagaaaaatatcgattctctaagtgcttaatccacatcactcaaagatttttataaccacaatattctaacttcaatcctgtattttaaaaaatccatagtgtaacatccatgaaagtatgttaaatcgttcctcttttacctacctcatcaaatagctactgaacattacccaaaggcatttattcgtaagtaatactgcttgatttacaaaattatttctcaaggaaaagttcaaaaggtggttatgtggatattcaaacaataccagaaaactcgctacttccttattcctgtaattaatgagtctggcttgcccagatgttaaattatgaaaccatgctgtgtaaaatgcacctattacaattaaaaccagggtaaacccgtatttatttactagcactgttaaaacattacacaaaacacattcaagtggcaagtaattataatgcaagcccttgcatggcaatccaaatttattgaactactgatgctaagttatacaaaattgcaccactttaattaaggcttttagtttacatttggccacctcaaagtagttgtaacattaggttggtcaatttaaatactgtggctccctgttggatagacacacaatctttacatccaaacattaatgcatacaaagcaacaaggcattgttaaataaaacagcaatagttactgcaaattaggccttgtgaccaattacatatgattaaaattacttcccacattcacatccacagtactcgtccaccatttaacatctcaaccaaaacgttacacatgtgaaacaatcactaacaggcaaaaatactaaacctgtatatttggtattgcaaatacacttatgcatgagcaagcaagggattcacagtgagaatctacagctgcagaagcctgaaaatgatttacaaaaattgttaaatcattaaaaaattgtttgaaaatatacacttcttgttgtagacccccactgtacacacgactataaacattgttccctatgtaaacaaaaaaaggaaacatataataagagatttgaaaagtctggacatttccttcccaacagatattaaaggcaacgtctttaatctaagacattatactgaaaggactatcatgttttaaagacaagatcaccgtctccacaggttttttaaaaattaaaaaaactatatagctgtgttaatcaaagcgcttattttgtacaataataatgaccttgaatttcttaaaaaaaattacaataagctacaagtatcaaagaagcgaagttatctggagtagtctatataggagctctttggactttcttttattatgctaaaatagtggtgcttttaggatttacattattgtactctccaatacaaagtatggggcatgttaaagtatacagtacaccattttcatacatgtacaacattggtggatgaagaatgtctcttagcagtaatactggatgtagcctctggttttaccagctgcaaactctaggactattatataagtaaaaatctctcttgtgatactggaaagtgattagaatgtgcaaactgatatagtagctttcatccgcctcttaaagggtaccaccacaggaaagtccatttaagatgttggtaggtttaacaaagttggaatgctggcactgttgaattgggcaacagttcttcagacctggctcagagctacaatgcatttagtatattaaagcagctgacatgatgactttttgcgagccttcccaggcactggagtttttctgttaatttgccgcactaggtcataaaagatctcattaacatttatttttgattttgcagaagattctaagaatgcacagttgttccattgtcttgctagattttgaccttgttccttccctacaactctttcatcttccaagtcacacttattaccaacaagaatcattggaacatcatcagtgtctttaactcgaagaatctgttctctcaggtcttgtaaatcgttaaatgtggactgtgctgtgatggaataaactaatgcaaatccttgtccatttttcatgtataaatccctcattgctgtaaattgctccaaagcagactttccaacgcctcctgagccaagaacgactagcttatactcacgcatgatgcaagcttgtcaaaacctagtactctgcgaacctctcacgctgtcaccgggtccctgcagccagcgtcgccccgcgctccccccgggtcgctactctaggcgccacggcggtcctgccgctgccgcgccgctccggctggtttacacgcctgaatctgggcgaggtttggcgatgtc

SEQ ID NO: 10851 - RNA, 4375 nt, Homo sapiens
  source 1..4375: mol_type = other RNA
ctgaatagctgggactacaggtacagacgtgcaccaccatgcccagctaattaaaaaaaaatttttttttgtagagatggggtctatgttgcccaggctgtcagatttgttttgtttgaaaaaaaaattttagtcttacaaatcacaatgttaaggctcactgacagattatgagacaagcctgcaagcacttttaaggcttctaaggtaatagtaagagtattaattgtaaaacactataactcccttttacatttccaagatttaagaagagatagaatagatggagattaaattcaatgaaaacacagataagagtttaactcaaagaaaagttgtagtgatgagtttcgattctaagtttgctgtcccacaactaaagacggaatgatttaaaaaaaaaaacggcaaaacttcattttataaatggaattttaaaaatttctatttgtaatgcccacatatggtaaagatgagctatttacgtttaagaaacaactgaatcaacaagaaagtcaatacagggtttttacactttttagaaaaatgtaagtgaaagaccactctgattttctcctaaaactcaagtttcttcaagtatccttggggacgtgaaaaggaattcatgccttttctgactcaattattttagtattttcccattaagcaccagaaaagtcaatctacatgagttgtgctcccaaactgcagttactattttgtataggagaaaatggtgctttttgccaaaccacagccttattcctatcagcattgaaaaaaataaattatatatatagtattatatagacctccactgtactacatatatatatatactctctctatatatgtactatatataatatatatatatatatatatatatagacctagaggatagcactggcattcatttcactctcctatgaagtaggtattatcattctcattttacagatgaggaaaccaaggcacccaaccaaaggcatatagtaggaactggaagagctgggattaaaaacccaggaagtctggctccaaactttatattcttattcactatatagtaaaccatccatcttgtaaccctaacactcatctgtaactaatgtgttgtttcccaccagagcagtagttcttcaccagggtgattttgccctccaagttcacctcccttgtcccccaacaatccaactggggaacatctggcaatgtctggaaacatttttggttgccacaacttgggggctggggtggtgtgactggcatctagtgggcagatattaaaattcctataatgcacaggagagtcgccagaatacattatcaaacataaaacatcaatagtgctgaggctgagaaactcttcaatagaatataaattctaggagggcagcattttatagttgatcttggttgctgctacatccttaggcctagaacaatttttatacttaagtacttaatttgtccaatgaatgaatatttagctgtttgagcctagaactgggcctggtacatagctggtaggcagcaaacatttattaaaagtaattattgaataatggcggtatcaatggatgtaacaggacatagtaaattgaagtaattttagtgtttcacagtcccagttttttgggcttaatttttttcccaaatgattataaataaaaccagttctgccaaaacaagtcccttttgtaaagaatcagactttttcttaacatgaaagcctttaaaaatgtatcattcaaacagcgtgtatttaggggattagcagatacccctctattagatattatcactgattaattgctccagtagctggcaaatactttcaaaaagttttttaagagctttacaatttttaaaaagttttaaaataattctataagaattcagttcttacagaattcaattatagcatatttaagaaaaatatcgattctctaagtgcttaatccacatcactcaaagatttttataaccacaatattctaacttcaatcctgtattttaaaaaatccatagtgtaacatccatgaaagtatgttaaatcgttcctcttttacctacctcatcaaatagctactgaacattacccaaaggcatttattcgtaagtaatactgcttgatttacaaaattatttctcaaggaaaagttcaaaaggtggttatgtggatattcaaacaataccagaaaactcgctacttccttattcctgtaattaatgagtctggcttgcccagatgttaaattatgaaaccatgctgtgtaaaatgcacctattacaattaaaaccagggtaaacccgtatttatttactagcactgttaaaacattacacaaaacacattcaagtggcaagtaattataatgcaagcccttgcatggcaatccaaatttattgaactactgatgctaagttatacaaaattgcaccactttaattaaggcttttagtttacatttggccacctcaaagtagttgtaacattaggttggtcaatttaaatactgtggctccctgttggatagacacacaatctttacatccaaacattaatgcatacaaagcaacaaggcattgttaaataaaacagcaatagttactgcaaattaggccttgtgaccaattacatatgattaaaattacttcccacattcacatccacagtactcgtccaccatttaacatctcaaccaaaacgttacacatgtgaaacaatcactaacaggcaaaaatactaaacctgtatatttggtattgcaaatacacttatgcatgagcaagcaagggattcacagtgagaatctacagctgcagaagcctgaaaatgatttacaaaaattgttaaatcattaaaaaattgtttgaaaatatacacttcttgttgtagacccccactgtacacacgactataaacattgttccctatgtaaacaaaaaaaggaaacatataataagagatttgaaaagtctggacatttccttcccaacagatattaaaggcaacgtctttaatctaagacattatactgaaaggactatcatgttttaaagacaagatcaccgtctccacaggttttttaaaaattaaaaaaactatatagctgtgttaatcaaagcgcttattttgtacaataataatgaccttgaatttcttaaaaaaaattacaataagctacaagtatcaaagaagcgaagttatctggagtagtctatataggagctctttggactttcttttattatgctaaaatagtggtgcttttaggatttacattattgtactctccaatacaaagtatggggcatgttaaagtatacagtacaccattttcatacatgtacaacattggtggatgaagaatgtctcttagcagtaatactggatgtagcctctggttttaccagctgcaaactctaggactattatataagtaaaaatctctcttgtgatactggaaagtgattagaatgtgcaaactgatatagtagctttcatccgcctcttaaagggtaccaccacaggaaagtccatttaagatgttggtaggtttaacaaagttggaatgctggcactgttgaattgggcaacagttcttcagacctggctcagagctacaatgcatttagtatattaaagcagctgacatgatgactttttgcgagccttcccaggcactggagtttttctgttaatttgccgcactaggtcataaaagatctcattaacatttatttttgattttgcagaagattctaagaatgcacagttgttccattgtcttgctagattttgaccttgttccttccctacaactctttcatcttccaagtcacacttattaccaacaagaatcattggaacatcatcagtgtctttaactcgaagaatctgttctctcaggtcttgtaaatcgttaaatgtggactgtgctgtgatggaataaactaatgcaaatccttgtccatttttcatgtataaatccctcattgctgtaaattgctccgttcctgcagtatccaagatttcaagcatacactgttgtgcatctacttcaacttgctttctataagaatcttctatcgtaggatcgtatttttctacaaaaattccttgaacaaattgtacagtcaaagcagactttccaacgcctcctgagccaagaacgactagcttatactcacgcatgatgcaagcttgtcaaaacctagtacctctcacgctgtcaccgggtccctgcagccagcgtcgccccgcgctccccccgggtcgctactctaggcgccacggcggtcctgccgctgccgcgccgctccggctggtttacacgcctgaatctgggcgaggtttggcgatgtc

SEQ ID NO: 10852 - RNA, 4384 nt, Homo sapiens
  source 1..4384: mol_type = other RNA
ctgaatagctgggactacaggtacagacgtgcaccaccatgcccagctaattaaaaaaaaatttttttttgtagagatggggtctatgttgcccaggctgtcagatttgttttgtttgaaaaaaaaattttagtcttacaaatcacaatgttaaggctcactgacagattatgagacaagcctgcaagcacttttaaggcttctaaggtaatagtaagagtattaattgtaaaacactataactcccttttacatttccaagatttaagaagagatagaatagatggagattaaattcaatgaaaacacagataagagtttaactcaaagaaaagttgtagtgatgagtttcgattctaagtttgctgtcccacaactaaagacggaatgatttaaaaaaaaaaacggcaaaacttcattttataaatggaattttaaaaatttctatttgtaatgcccacatatggtaaagatgagctatttacgtttaagaaacaactgaatcaacaagaaagtcaatacagggtttttacactttttagaaaaatgtaagtgaaagaccactctgattttctcctaaaactcaagtttcttcaagtatccttggggacgtgaaaaggaattcatgccttttctgactcaattattttagtattttcccattaagcaccagaaaagtcaatctacatgagttgtgctcccaaactgcagttactattttgtataggagaaaatggtgctttttgccaaaccacagccttattcctatcagcattgaaaaaaataaattatatatatagtattatatagacctccactgtactacatatatatatatactctctctatatatgtactatatataatatatatatatatatatatatatagacctagaggatagcactggcattcatttcactctcctatgaagtaggtattatcattctcattttacagatgaggaaaccaaggcacccaaccaaaggcatatagtaggaactggaagagctgggattaaaaacccaggaagtctggctccaaactttatattcttattcactatatagtaaaccatccatcttgtaaccctaacactcatctgtaactaatgtgttgtttcccaccagagcagtagttcttcaccagggtgattttgccctccaagttcacctcccttgtcccccaacaatccaactggggaacatctggcaatgtctggaaacatttttggttgccacaacttgggggctggggtggtgtgactggcatctagtgggcagatattaaaattcctataatgcacaggagagtcgccagaatacattatcaaacataaaacatcaatagtgctgaggctgagaaactcttcaatagaatataaattctaggagggcagcattttatagttgatcttggttgctgctacatccttaggcctagaacaatttttatacttaagtacttaatttgtccaatgaatgaatatttagctgtttgagcctagaactgggcctggtacatagctggtaggcagcaaacatttattaaaagtaattattgaataatggcggtatcaatggatgtaacaggacatagtaaattgaagtaattttagtgtttcacagtcccagttttttgggcttaatttttttcccaaatgattataaataaaaccagttctgccaaaacaagtcccttttgtaaagaatcagactttttcttaacatgaaagcctttaaaaatgtatcattcaaacagcgtgtatttaggggattagcagatacccctctattagatattatcactgattaattgctccagtagctggcaaatactttcaaaaagttttttaagagctttacaatttttaaaaagttttaaaataattctataagaattcagttcttacagaattcaattatagcatatttaagaaaaatatcgattctctaagtgcttaatccacatcactcaaagatttttataaccacaatattctaacttcaatcctgtattttaaaaaatccatagtgtaacatccatgaaagtatgttaaatcgttcctcttttacctacctcatcaaatagctactgaacattacccaaaggcatttattcgtaagtaatactgcttgatttacaaaattatttctcaaggaaaagttcaaaaggtggttatgtggatattcaaacaataccagaaaactcgctacttccttattcctgtaattaatgagtctggcttgcccagatgttaaattatgaaaccatgctgtgtaaaatgcacctattacaattaaaaccagggtaaacccgtatttatttactagcactgttaaaacattacacaaaacacattcaagtggcaagtaattataatgcaagcccttgcatggcaatccaaatttattgaactactgatgctaagttatacaaaattgcaccactttaattaaggcttttagtttacatttggccacctcaaagtagttgtaacattaggttggtcaatttaaatactgtggctccctgttggatagacacacaatctttacatccaaacattaatgcatacaaagcaacaaggcattgttaaataaaacagcaatagttactgcaaattaggccttgtgaccaattacatatgattaaaattacttcccacattcacatccacagtactcgtccaccatttaacatctcaaccaaaacgttacacatgtgaaacaatcactaacaggcaaaaatactaaacctgtatatttggtattgcaaatacacttatgcatgagcaagcaagggattcacagtgagaatctacagctgcagaagcctgaaaatgatttacaaaaattgttaaatcattaaaaaattgtttgaaaatatacacttcttgttgtagacccccactgtacacacgactataaacattgttccctatgtaaacaaaaaaaggaaacatataataagagatttgaaaagtctggacatttccttcccaacagatattaaaggcaacgtctttaatctaagacattatactgaaaggactatcatgttttaaagacaagatcaccgtctccacaggttttttaaaaattaaaaaaactatatagctgtgttaatcaaagcgcttattttgtacaataataatgaccttgaatttcttaaaaaaaattacaataagctacaagtatcaaagaagcgaagttatctggagtagtctatataggagctctttggactttcttttattatgctaaaatagtggtgcttttaggatttacattattgtactctccaatacaaagtatggggcatgttaaagtatacagtacaccattttcatacatgtacaacattggtggatgaagaatgtctcttagcagtaatactggatgtagcctctggttttaccagctgcaaactctaggactattatataagtaaaaatctctcttgtgatactggaaagtgattagaatgtgcaaactgatatagtagctttcatccgcctcttaaagggtaccaccacaggaaagtccatttaagatgttggtaggtttaacaaagttggaatgctggcactgttgaattgggcaacagttcttcagacctggctcagagctacaatgcatttagtatattaaagcagctgacatgatgactttttgcgagccttcccaggcactggagtttttctgttaatttgccgcactaggtcataaaagatctcattaacatttatttttgattttgcagaagattctaagaatgcacagttgttccattgtcttgctagattttgaccttgttccttccctacaactctttcatcttccaagtcacacttattaccaacaagaatcattggaacatcatcagtgtctttaactcgaagaatctgttctctcaggtcttgtaaatcgttaaatgtggactgtgctgtgatggaataaactaatgcaaatccttgtccatttttcatgtataaatccctcattgctgtaaattgctccgttcctgcagtatccaagatttcaagcatacactgttgtgcatctacttcaacttgctttctataagaatcttctatcgtaggatcgtatttttctacaaaaattccttgaacaaattgtacagtcaaagcagactttccaacgcctcctgagccaagaacgactagcttatactcacgcatgatgcaagcttgtcaaaacctagtactctgcgaacctctcacgctgtcaccgggtccctgcagccagcgtcgccccgcgctccccccgggtcgctactctaggcgccacggcggtcctgccgctgccgcgccgctccggctggtttacacgcctgaatctgggcgaggtttggcgatgtc

SEQ ID NO: 10853 - RNA, 4318 nt, Homo sapiens
  source 1..4318: mol_type = other RNA
ctgaatagctgggactacaggtacagacgtgcaccaccatgcccagctaattaaaaaaaaatttttttttgtagagatggggtctatgttgcccaggctgtcagatttgttttgtttgaaaaaaaaattttagtcttacaaatcacaatgttaaggctcactgacagattatgagacaagcctgcaagcacttttaaggcttctaaggtaatagtaagagtattaattgtaaaacactataactcccttttacatttccaagatttaagaagagatagaatagatggagattaaattcaatgaaaacacagataagagtttaactcaaagaaaagttgtagtgatgagtttcgattctaagtttgctgtcccacaactaaagacggaatgatttaaaaaaaaaaacggcaaaacttcattttataaatggaattttaaaaatttctatttgtaatgcccacatatggtaaagatgagctatttacgtttaagaaacaactgaatcaacaagaaagtcaatacagggtttttacactttttagaaaaatgtaagtgaaagaccactctgattttctcctaaaactcaagtttcttcaagtatccttggggacgtgaaaaggaattcatgccttttctgactcaattattttagtattttcccattaagcaccagaaaagtcaatctacatgagttgtgctcccaaactgcagttactattttgtataggagaaaatggtgctttttgccaaaccacagccttattcctatcagcattgaaaaaaataaattatatatatagtattatatagacctccactgtactacatatatatatatactctctctatatatgtactatatataatatatatatatatatatatatatagacctagaggatagcactggcattcatttcactctcctatgaagtaggtattatcattctcattttacagatgaggaaaccaaggcacccaaccaaaggcatatagtaggaactggaagagctgggattaaaaacccaggaagtctggctccaaactttatattcttattcactatatagtaaaccatccatcttgtaaccctaacactcatctgtaactaatgtgttgtttcccaccagagcagtagttcttcaccagggtgattttgccctccaagttcacctcccttgtcccccaacaatccaactggggaacatctggcaatgtctggaaacatttttggttgccacaacttgggggctggggtggtgtgactggcatctagtgggcagatattaaaattcctataatgcacaggagagtcgccagaatacattatcaaacataaaacatcaatagtgctgaggctgagaaactcttcaatagaatataaattctaggagggcagcattttatagttgatcttggttgctgctacatccttaggcctagaacaatttttatacttaagtacttaatttgtccaatgaatgaatatttagctgtttgagcctagaactgggcctggtacatagctggtaggcagcaaacatttattaaaagtaattattgaataatggcggtatcaatggatgtaacaggacatagtaaattgaagtaattttagtgtttcacagtcccagttttttgggcttaatttttttcccaaatgattataaataaaaccagttctgccaaaacaagtcccttttgtaaagaatcagactttttcttaacatgaaagcctttaaaaatgtatcattcaaacagcgtgtatttaggggattagcagatacccctctattagatattatcactgattaattgctccagtagctggcaaatactttcaaaaagttttttaagagctttacaatttttaaaaagttttaaaataattctataagaattcagttcttacagaattcaattatagcatatttaagaaaaatatcgattctctaagtgcttaatccacatcactcaaagatttttataaccacaatattctaacttcaatcctgtattttaaaaaatccatagtgtaacatccatgaaagtatgttaaatcgttcctcttttacctacctcatcaaatagctactgaacattacccaaaggcatttattcgtaagtaatactgcttgatttacaaaattatttctcaaggaaaagttcaaaaggtggttatgtggatattcaaacaataccagaaaactcgctacttccttattcctgtaattaatgagtctggcttgcccagatgttaaattatgaaaccatgctgtgtaaaatgcacctattacaattaaaaccagggtaaacccgtatttatttactagcactgttaaaacattacacaaaacacattcaagtggcaagtaattataatgcaagcccttgcatggcaatccaaatttattgaactactgatgctaagttatacaaaattgcaccactttaattaaggcttttagtttacatttggccacctcaaagtagttgtaacattaggttggtcaatttaaatactgtggctccctgttggatagacacacaatctttacatccaaacattaatgcatacaaagcaacaaggcattgttaaataaaacagcaatagttactgcaaattaggccttgtgaccaattacatatgattaaaattacttcccacattcacatccacagtactcgtccaccatttaacatctcaaccaaaacgttacacatgtgaaacaatcactaacaggcaaaaatactaaacctgtatatttggtattgcaaatacacttatgcatgagcaagcaagggattcacagtgagaatctacagctgcagaagcctgaaaatgatttacaaaaattgttaaatcattaaaaaattgtttgaaaatatacacttcttgttgtagacccccactgtacacacgactataaacattgttccctatgtaaacaaaaaaaggaaacatataataagagatttgaaaagtctggacatttccttcccaacagatattaaaggcaacgtctttaatctaagacattatactgaaaggactatcatgttttaaagacaagatcaccgtctccacaggttttttaaaaattaaaaaaactatatagctgtgttaatcaaagcgcttattttgtacaataataatgaccttgaatttcttaaaaaaaattacaataagctacaagtatcaaagaagcgaagttatctggagtagtctatataggagctctttggactttcttttattatgctaaaatagtggtgcttttaggatttacattattgtactctccaatacaaagtatggggcatgttaaagtatacagtacaccattttcatacatgtacaacattggtggatgaagaatgtctcttagcagtaatactggatgtagcctctggttttaccagctgcaaactctaggactattatataagtaaaaatctctcttgtgatactggaaagtgattagaatgtgcaaactgatatagtagctttcatccgcctcttaaagggtaccaccacaggaaagtccatttaagatgttggtaggtttaacaaagttggaatgctggcactgttgaattgggcaacagttcttcagacctggctcagagctacaatgcatttagtatattaaagcagctgacatgatgactttttgcgagccttcccaggcactggagtttttctgttaatttgccgcactaggtcataaaagatctcattaacatttatttttgattttgcagaagattctaagaatgcacagttgttccattgtcttgctagattttgaccttgttccttccctacaactctttcatcttccaagtcacacttattaccaacaagaatcattggaacatcatcagtgtctttaactcgaagaatctgttctctcaggtcttgtaaatcgttaaatgtggactgtgctgtgatggaataaactaatgcaaatccttgtccatttttcatgtataaatccctcattgctgtaaattgctcctttctataagaatcttctatcgtaggatcgtatttttctacaaaaattccttgaacaaattgtacagtcaaagcagactttccaacgcctcctgagccaagaacgactagcttatactcacgcatgatgcaagcttgtcaaaacctagtacctctcacgctgtcaccgggtccctgcagccagcgtcgccccgcgctccccccgggtcgctactctaggcgccacggcggtcctgccgctgccgcgccgctccggctggtttacacgcctgaatctgggcgaggtttggcgatgtc

SEQ ID NO: 10854 - RNA, 4234 nt, Homo sapiens
  source 1..4234: mol_type = other RNA
ctgaatagctgggactacaggtacagacgtgcaccaccatgcccagctaattaaaaaaaaatttttttttgtagagatggggtctatgttgcccaggctgtcagatttgttttgtttgaaaaaaaaattttagtcttacaaatcacaatgttaaggctcactgacagattatgagacaagcctgcaagcacttttaaggcttctaaggtaatagtaagagtattaattgtaaaacactataactcccttttacatttccaagatttaagaagagatagaatagatggagattaaattcaatgaaaacacagataagagtttaactcaaagaaaagttgtagtgatgagtttcgattctaagtttgctgtcccacaactaaagacggaatgatttaaaaaaaaaaacggcaaaacttcattttataaatggaattttaaaaatttctatttgtaatgcccacatatggtaaagatgagctatttacgtttaagaaacaactgaatcaacaagaaagtcaatacagggtttttacactttttagaaaaatgtaagtgaaagaccactctgattttctcctaaaactcaagtttcttcaagtatccttggggacgtgaaaaggaattcatgccttttctgactcaattattttagtattttcccattaagcaccagaaaagtcaatctacatgagttgtgctcccaaactgcagttactattttgtataggagaaaatggtgctttttgccaaaccacagccttattcctatcagcattgaaaaaaataaattatatatatagtattatatagacctccactgtactacatatatatatatactctctctatatatgtactatatataatatatatatatatatatatatatagacctagaggatagcactggcattcatttcactctcctatgaagtaggtattatcattctcattttacagatgaggaaaccaaggcacccaaccaaaggcatatagtaggaactggaagagctgggattaaaaacccaggaagtctggctccaaactttatattcttattcactatatagtaaaccatccatcttgtaaccctaacactcatctgtaactaatgtgttgtttcccaccagagcagtagttcttcaccagggtgattttgccctccaagttcacctcccttgtcccccaacaatccaactggggaacatctggcaatgtctggaaacatttttggttgccacaacttgggggctggggtggtgtgactggcatctagtgggcagatattaaaattcctataatgcacaggagagtcgccagaatacattatcaaacataaaacatcaatagtgctgaggctgagaaactcttcaatagaatataaattctaggagggcagcattttatagttgatcttggttgctgctacatccttaggcctagaacaatttttatacttaagtacttaatttgtccaatgaatgaatatttagctgtttgagcctagaactgggcctggtacatagctggtaggcagcaaacatttattaaaagtaattattgaataatggcggtatcaatggatgtaacaggacatagtaaattgaagtaattttagtgtttcacagtcccagttttttgggcttaatttttttcccaaatgattataaataaaaccagttctgccaaaacaagtcccttttgtaaagaatcagactttttcttaacatgaaagcctttaaaaatgtatcattcaaacagcgtgtatttaggggattagcagatacccctctattagatattatcactgattaattgctccagtagctggcaaatactttcaaaaagttttttaagagctttacaatttttaaaaagttttaaaataattctataagaattcagttcttacagaattcaattatagcatatttaagaaaaatatcgattctctaagtgcttaatccacatcactcaaagatttttataaccacaatattctaacttcaatcctgtattttaaaaaatccatagtgtaacatccatgaaagtatgttaaatcgttcctcttttacctacctcatcaaatagctactgaacattacccaaaggcatttattcgtaagtaatactgcttgatttacaaaattatttctcaaggaaaagttcaaaaggtggttatgtggatattcaaacaataccagaaaactcgctacttccttattcctgtaattaatgagtctggcttgcccagatgttaaattatgaaaccatgctgtgtaaaatgcacctattacaattaaaaccagggtaaacccgtatttatttactagcactgttaaaacattacacaaaacacattcaagtggcaagtaattataatgcaagcccttgcatggcaatccaaatttattgaactactgatgctaagttatacaaaattgcaccactttaattaaggcttttagtttacatttggccacctcaaagtagttgtaacattaggttggtcaatttaaatactgtggctccctgttggatagacacacaatctttacatccaaacattaatgcatacaaagcaacaaggcattgttaaataaaacagcaatagttactgcaaattaggccttgtgaccaattacatatgattaaaattacttcccacattcacatccacagtactcgtccaccatttaacatctcaaccaaaacgttacacatgtgaaacaatcactaacaggcaaaaatactaaacctgtatatttggtattgcaaatacacttatgcatgagcaagcaagggattcacagtgagaatctacagctgcagaagcctgaaaatgatttacaaaaattgttaaatcattaaaaaattgtttgaaaatatacacttcttgttgtagacccccactgtacacacgactataaacattgttccctatgtaaacaaaaaaaggaaacatataataagagatttgaaaagtctggacatttccttcccaacagatattaaaggcaacgtctttaatctaagacattatactgaaaggactatcatgttttaaagacaagatcaccgtctccacaggttttttaaaaattaaaaaaactatatagctgtgttaatcaaagcgcttattttgtacaataataatgaccttgaatttcttaaaaaaaattacaataagctacaagtatcaaagaagcgaagttatctggagtagtctatataggagctctttggactttcttttattatgctaaaatagtggtgcttttaggatttacattattgtactctccaatacaaagtatggggcatgttaaagtatacagtacaccattttcatacatgtacaacattggtggatgaagaatgtctcttagcagtaatactggatgtagcctctggttttaccagctgcaaactctaggactattatataagtaaaaatctctcttgtgatactggaaagtgattagaatgtgcaaactgatatagtagctttcatccgcctcttaaagggtaccaccacaggaaagtccatttaagatgttggtaggtttaacaaagttggaatgctggcactgttgaattgggcaacagttcttcagacctggctcagagctacaatgcatttagtatattaaagcagctgacatgatgactttttgcgagccttcccaggcactggagtttttctgttaatttgccgcactaggtcataaaagatctcattaacatttatttttgattttgcagaagattctaagaatgcacagttgttccattgtcttgctagattttgaccttgttccttccctacaactctttcatcttccaagtcacacttattaccaacaagaatcattggaaccgttcctgcagtatccaagatttcaagcatacactgttgtgcatctacttcaacttgctttctataagaatcttctatcgtaggatcgtatttttctacaaaaattccttgaacaaattgtacagtcaaagcagactttccaacgcctcctgagccaagaacgactagcttatactcacgcatgatgcaagcttgtcaaaacctagtacctctcacgctgtcaccgggtccctgcagccagcgtcgccccgcgctccccccgggtcgctactctaggcgccacggcggtcctgccgctgccgcgccgctccggctggtttacacgcctgaatctgggcgaggtttggcgatgtc

SEQ ID NO: 10855 - RNA, 1306 nt, Homo sapiens
  source 1..1306: mol_type = other RNA
ctgaatagctgggactacaggtacatgccaccgcacccggctaatttttttatttttagtacacacgaggtttcaccatattggccaggctggtctcgaactcctgacctcgtgatccgcccgccttggcctcccaaagtgctgggattacatgcgtgagccgccgcacccagcccctgaattacctatgactttatcaagggaaagagtcacctgtgttgttaaagctgagctgatgacagctccacaaatgttaactgaacaaagtgccacactatgtgcctgtgtctgaagatgaatgagacacaatctgtgtgttctcggagcttctccaaggtgaacttttctggggcttaacctgcaactggccaggaacagcagcttaaaatctcatcaatagctgtgctatttcaaagtactggcattctcccaggacatcccccagggtgtcaaaatttagccaaagcaaacttcaaatgaacacaaagtccttattttctcaaagaaaacaaaacaaaacagaacaaaaaaccccccagatttatttagcttaaacatttcccctgatctaaagagaaagatggcaaaagatacctagcatatatgcacaagcacccactccaatgaactcagataacctgaaagaaaaaaggacaaagttctgttcaacttagaaaattatcttcgcttttgaaagatgtttccacgtcccattccacgtcctcttcctcttgcggccactggcagttcatgttgtcctctgcttcaatgagcttcccccgatatacctcaccggtgttcgtctcacatgtcacaatgtggccctcggcctcatgcagtactttaatcggcacaccaatagacatcttggcaggaagagagttcggctctggcctacttttcttctcttcggtccgctgcgaaagatgctacggcgaaggcgtgagtcaagcgaatggcgggcctaacacccagaattccactctttcccaaaatgctgcgcgcagggcccgcctccttcctttccccagtgttgagcgcggtctcgcctccgcttcctcctcactccgcctgccggctgggaaactagggcaccagtacgatagttccggcaccggaaaagagggctgatgactgggcccgggggccgccgcaacgacccttggggccggcaaagagccagagagggtgctcacacttccaagcaccccacaccaaggacaggctggacggcaaggcggagacgcggggcttgggccctcagaccggggacagcaggaggttgggccaagggccaggacttccc

SEQ ID NO: 10856 - RNA, 1150 nt, Homo sapiens
  source 1..1150: mol_type = other RNA
ctgaatagctgggactacaggtacatgccaccgcacccggctaatttttttatttttagtacacacgaggtttcaccatattggccaggctggtctcgaactcctgacctcgtgatccgcccgccttggcctcccaaagtgctgggattacatgcgtgagccgccgcacccagcccctgaattacctatgactttatcaagggaaagagtcacctgtgttgttaaagctgagctgatgacagctccacaaatgttaactgaacaaagtgccacactatgtgcctgtgtctgaagatgaatgagacacaatctgtgtgttctcggagcttctccaaggtgaacttttctggggcttaacctgcaactggccaggaacagcagcttaaaatctcatcaatagctgtgctatttcaaagtactggcattctcccaggacatcccccagggtgtcaaaatttagccaaagcaaacttcaaatgaacacaaagtccttattttctcaaagaaaacaaaacaaaacagaacaaaaaaccccccagatttatttagcttaaacatttcccctgatctaaagagaaagatggcaaaagatacctagcatatatgcacaagcacccactccaatgaactcagataacctgaaagaaaaaaggacaaagttctgttcaacttagaaaattatcttcgcttttgaaagatgtttccacgtcccattccacgtcctcttcctcttgcggccacttgggccttgagaatagcagcttttcctcggccagcccctgagccttggtttttatttttcatgctctttaacatgggtgcgttcttcagcatgtcaggcaaaatcagaaagcggattttgctgccacggatgtatacctgctccagctgtgccactcggccatctctgtatgtgactgtgatgttggacatctggcagttcatgttgtcctctgcttcaatgagcttcccccgatatacctcaccggtgttcgtctcacatgtcacaatgtggccctcggcctcatgcagtactttaatcggcacaccaatagacatcttggcaggaagagagttcggctctggcctacttttcttctcttcggtccgctgcgaaagatgctacggcgaaggcgtgagtcaagcgaat

SEQ ID NO: 10857 - RNA, 1136 nt, Homo sapiens
  source 1..1136: mol_type = other RNA
ctgaatagctgggactacaggtacatgccaccgcacccggctaatttttttatttttagtacacacgaggtttcaccatattggccaggctggtctcgaactcctgacctcgtgatccgcccgccttggcctcccaaagtgctgggattacatgcgtgagccgccgcacccagcccctgaattacctatgactttatcaagggaaagagtcacctgtgttgttaaagctgagctgatgacagctccacaaatgttaactgaacaaagtgccacactatgtgcctgtgtctgaagatgaatgagacacaatctgtgtgttctcggagcttctccaaggtgaacttttctggggcttaacctgcaactggccaggaacagcagcttaaaatctcatcaatagctgtgctatttcaaagtactggcattctcccaggacatcccccagggtgtcaaaatttagccaaagcaaacttcaaatgaacacaaagtccttattttctcaaagaaaacaaaacaaaacagaacaaaaaaccccccagatttatttagcttaaacatttcccctgatctaaagagaaagatggcaaaagatacctagcatatatgcacaagcacccactccaatgaactcagataacctgaaagaaaaaaggacaaagttctgttcaacttagaaaattatcttcgcttttgaaagatgtttccacgtcccattccacgtcctcttcctcttgcggccacttgggccttgagaatagcagcttttcctcggccagcccctgagccttggtttttatttttcatgctctttaacatgggtgcgttcttcagcatgtcaggcaaaatcagaaagcggattttgctgccacggatgtatacctgctccagctgtgccactcggccatctctgtatgtgactgtgatgttggacatctggcagttcatgttgtcctctgcttcaatgagcttcccccgatatacctcaccggtgttcgtctcacatgtcacaatgtggccctcggcctcatgcagtactttaatcggcacaccaatagacatcttggcaggaagagagttttttcttctcttcggtccgctgcgaaagatgctacggcgaaggcgtgagtcaagcgaat

SEQ ID NO: 10858 - RNA, 4697 nt, Homo sapiens
  source 1..4697: mol_type = other RNA
ctgaatagctgggactacaggtacattgctaattttttaaaaattagccgggggggcggggggtctcttttgaaattagatggtggtctctccatgttgccagactggtcttgaacttctggtatcaagtgatcctcccgccttggcctcccaaagtgctgagattacaggtgtgagtcactgcacccagccctaaatcataccatttagagtcatgattgttggagaattttgaaaacatctgcattgtagaaacctttcccctcccctccctgacccttgctcctgtcatgtaccagtgtacttcctggacatcaaagtgcctgctgcatatgtccaactcactggctgggagggtgcttcagcagcaacacacatcaagggcaggtctccttgaagccaacagaagtaagaggaaggggctgagaatcagtgccagttgggtggggggacacctggcctctccctctctcggcaccagcttttcccaaggtctgatcagaatgtttcctttctactgccatgtccattttttcatggtattttaatttccttctttatcctggaaaagacattggagaatccccttcccccaagttaaataagacaaggttggagtttttcaaaaggagcatttactaggaaactaaagggcaaccaaacagaatgcaagagaacagaggcagagttgcaaatgggctgagggagttcaaatttataaccagcctctgctcacagctgtactggctaggcaaagctttccagacacaaagccacctgcctgccatgtggatagtactctttgcctgcttgcccctacaaagccaccttctatttcataccaataagccagttgcatcctcattagtatcccaaggctgctggctctctgggcaggaagcttctgaggtggggaacagtaggcacagctgcctcaggatctccaacccaggcttccattgccaaggacatgtcagaatttattgggattgctgcctgatatctattggagccagtctgctttctctgggaccattcttctgggctcatctgcctagctttacagacaatatttctgctaactatcctggtggcgctagcccttcatgttttgcttctaaacactggtatggtggaggatgtctgaatgaggagggatgagcagaggggaaccttgagcagaggaagccaagttttccttatgtcatcagacataggcagaaccttggattctctttgaatcccagtggttggaagccaatcagagaagtgaagcttgaatgtaatgacactgcttcctacaaacaaaggcctatagccttcttagatctgccatcaaagtagagcttcttgtatagtactaggcagctggggcaatgagaactttctgaagacgtataacgatccttcctccgcccagttagttccatgctgaaatgttaattcaaacagagataatgagctttccaggaaggtaaactacaatccaactctggattctgctgtaaagagattgtgtgaaaagaaaaatactatcttggagtagtggtgcaaatgtgtggatggggtgccttgcacctataatgggacagagaggaccattaggtaacagcccccagtcctcccaggatatgctgaggcctttggtttcatttacgtggaggcagaagcaatgaggatgaggcgcatagctggccattggttggcagacttggtcaggaaggaagctgagtaatgaatgagatgcctggggagggcccttgaccttcactcttgtaggtatttccatccccaagtggtgtgaaagtgatgtatgtgtctgaagtgagaaggaaacctctatgtgtggttgcccaaggctatgactctgggctgttgcatatggaaataccccagaaggcattcaggccagagaagcccaaaagctgtgcctttctataggggatggctgtgttctctctccatgatctcatctcacccattgctgtaccagtttctgaggctgttcccttagtggacgaatgtgcctaggaaaggatattccacaatgctcatgccactgagatgtatgcccttctaactaattacttttcattctaataacactcccagttgaaaggaaggggctgctagctactgagtgagtagtgttgggggtctctgattcctcaaaatctggttttagcagaaaacagggccatgttgatactggtactctctaccacgtgcatgggaggaggcagtgaatttgctgtgaactagccctccttgcattagattttttccagggaacagcctgcttgtcttggtattctcttggggctattccttgcaaatctggagcacttcttggggcacagttattttctggagacagtcattagctcaaaggtagtcatgtgtgaattgagatctgctgcctatttagcacctggatatatttttaaatattctgtccttccagggcattctagaaaataatattatgttggaataacgatttccagggcagatgctatgtcctcatcaccaagggcttcatatgaaacattgagtcctggtactcttggtactgtcactatatctatcatttgtttttgttcatagtccgatcttggttcttggcatgagagacatgcttccctgcagcacatcaccttgggccacctgcagaaggtggctggaccattcaggttcaccaaacccaatctggaaagaaggccagttagtgctgtggttacagctgagcatttggtcactgaaatcgtctggatgttgctggatggaaaaagttacttaagatctttgtgagatggttgtcctattttgtccttggcacaagcagtcctcttacccatggtcatcgtttcccgaaccaatccctgaatgtgatgattgggcttaagcctggggagatgcaaagacattcctggagctgaggatgtggatgcctctacccaaaccacatggttagagggggaagaggggtgagtcctcaaaggaaaatgtggttcttttatctccaccagggaatgccagtgtgcaatgggcttccgaggatatgacaacatttcactccagtggtctctgcccagcctctcagcctcgttgcctacttgacacacgccgatgatctcattgtgaccggtcatagtccatgactgctatggacaagtggatttggtcaatgttctcgggagggacatcaaagactatggcttcgttgtaaacaggattcaaggtgttcctcttggtggatgttttcctcttcttcagtcgtctgccatcacacatcagcgagactttcacatagggatctgatgctcctgttatgtccattgcctttaaattccttgcttttataatggtaatggtcagcctgccagccgttggaagatagcacagggaaaacatcagctctcccagatccacgttgtcattggtgacatattcgatatccttccaaaggatgcactccctggggaaatcagccaagtctaggaagtgatccaccaccacttggccgattaagtcatgacgagagaacctgtcaaagtcgtacacagagaagtgaagcttccgtgcttcaaggtcattgtagggaaccggaaataaaaacacttcatcaaacacagggttcagggtctttctgtgaactttagtctggtgttttgttttccgatcaggaagcaaatagatcttgacataaggatctgaagtcccagaaaagtccttggcgggcaaattgacagctttgtgaatcttcactatgagctgctctaagtcacagtcatattttaaaatgaagttcagtttcccacaagccttgctgttactccgtctcccgtcatcattatccaatgacctctgcttatataactctggtttaattctaccaattccagtcaactgttcctgtttttgaagctgctggatattgaagtccgggtttgacaagttgagttgtcttcggattgaattatgccgggccgacgaggttggctctgtgacttggcgctgcacgcggacgccatgggcacagttctcctggatccccgtctgggtggagaggggaatgtcaggggaggtgtggctgatcttcatggaggagtcagggcagggcgtgggaggatctaggaagtcctcactgttctcctgctcattggtctctgtgtccatgtagttaaggggctcctggttgttgtctttgctaccagagggcaggcctcgttctcgccacggaacccagcagagtttccaagatacgaagagagacacgccaaagagagcgagaccacaggcagtgaccacaagggtcagcaggctcactgagatatctgggtcgcggagccggggtctggcacggtcccgcaggtggtaaatgaaatcctggcagctgtcgtgctccagggccccacgggcacagagctcggccagcagctgcagcgcctggtgacagagcgcgtccctggccccgggcatcgcccccccgcatcctcggaccgcgccgggcaggcgggcgcaggagacagccctccgcctgccagctcagagccgccgcctccgggccgtccgcgctcaccgccagggacctgccgagaaacggtgcgagcctgagcccgagccccagacccagccggcccggcctcccaccggttgcatgcagctcttcgccagccggtcggtcaggctttctc

SEQ ID NO: 10859 - RNA, 4702 nt, Homo sapiens
  source 1..4702: mol_type = other RNA
ctgaatagctgggactacaggtacattgctaattttttaaaaattagccgggggggcggggggtctcttttgaaattagatggtggtctctccatgttgccagactggtcttgaacttctggtatcaagtgatcctcccgccttggcctcccaaagtgctgagattacaggtgtgagtcactgcacccagccctaaatcataccatttagagtcatgattgttggagaattttgaaaacatctgcattgtagaaacctttcccctcccctccctgacccttgctcctgtcatgtaccagtgtacttcctggacatcaaagtgcctgctgcatatgtccaactcactggctgggagggtgcttcagcagcaacacacatcaagggcaggtctccttgaagccaacagaagtaagaggaaggggctgagaatcagtgccagttgggtggggggacacctggcctctccctctctcggcaccagcttttcccaaggtctgatcagaatgtttcctttctactgccatgtccattttttcatggtattttaatttccttctttatcctggaaaagacattggagaatccccttcccccaagttaaataagacaaggttggagtttttcaaaaggagcatttactaggaaactaaagggcaaccaaacagaatgcaagagaacagaggcagagttgcaaatgggctgagggagttcaaatttataaccagcctctgctcacagctgtactggctaggcaaagctttccagacacaaagccacctgcctgccatgtggatagtactctttgcctgcttgcccctacaaagccaccttctatttcataccaataagccagttgcatcctcattagtatcccaaggctgctggctctctgggcaggaagcttctgaggtggggaacagtaggcacagctgcctcaggatctccaacccaggcttccattgccaaggacatgtcagaatttattgggattgctgcctgatatctattggagccagtctgctttctctgggaccattcttctgggctcatctgcctagctttacagacaatatttctgctaactatcctggtggcgctagcccttcatgttttgcttctaaacactggtatggtggaggatgtctgaatgaggagggatgagcagaggggaaccttgagcagaggaagccaagttttccttatgtcatcagacataggcagaaccttggattctctttgaatcccagtggttggaagccaatcagagaagtgaagcttgaatgtaatgacactgcttcctacaaacaaaggcctatagccttcttagatctgccatcaaagtagagcttcttgtatagtactaggcagctggggcaatgagaactttctgaagacgtataacgatccttcctccgcccagttagttccatgctgaaatgttaattcaaacagagataatgagctttccaggaaggtaaactacaatccaactctggattctgctgtaaagagattgtgtgaaaagaaaaatactatcttggagtagtggtgcaaatgtgtggatggggtgccttgcacctataatgggacagagaggaccattaggtaacagcccccagtcctcccaggatatgctgaggcctttggtttcatttacgtggaggcagaagcaatgaggatgaggcgcatagctggccattggttggcagacttggtcaggaaggaagctgagtaatgaatgagatgcctggggagggcccttgaccttcactcttgtaggtatttccatccccaagtggtgtgaaagtgatgtatgtgtctgaagtgagaaggaaacctctatgtgtggttgcccaaggctatgactctgggctgttgcatatggaaataccccagaaggcattcaggccagagaagcccaaaagctgtgcctttctataggggatggctgtgttctctctccatgatctcatctcacccattgctgtaccagtttctgaggctgttcccttagtggacgaatgtgcctaggaaaggatattccacaatgctcatgccactgagatgtatgcccttctaactaattacttttcattctaataacactcccagttgaaaggaaggggctgctagctactgagtgagtagtgttgggggtctctgattcctcaaaatctggttttagcagaaaacagggccatgttgatactggtactctctaccacgtgcatgggaggaggcagtgaatttgctgtgaactagccctccttgcattagattttttccagggaacagcctgcttgtcttggtattctcttggggctattccttgcaaatctggagcacttcttggggcacagttattttctggagacagtcattagctcaaaggtagtcatgtgtgaattgagatctgctgcctatttagcacctggatatatttttaaatattctgtccttccagggcattctagaaaataatattatgttggaataacgatttccagggcagatgctatgtcctcatcaccaagggcttcatatgaaacattgagtcctggtactcttggtactgtcactatatctatcatttgtttttgttcatagtccgatcttggttcttggcatgagagacatgcttccctgcagcacatcaccttgggccacctgcagaaggtggctggaccattcaggttcaccaaacccaatctggaaagaaggccagttagtgctgtggttacagctgagcatttggtcactgaaatcgtctggatgttgctggatggaaaaagttacttaagatctttgtgagatggttgtcctattttgtccttggcacaagcagtcctcttacccatggtcatcgtttcccgaaccaatccctgaatgtgatgattgggcttaagcctggggagatgcaaagacattcctggagctgaggatgtggatgcctctacccaaaccacatggttagagggggaagaggggtgagtcctcaaaggaaaatgtggttcttttatctccaccagggaatgccagtgtgcaatgggcttccgaggatatgacaacatttcactccagtggtctctgcccagcctctcagcctcgttgcctacttgacacacgccgatgatctcattgtgacctacacggtcatagtccatgactgctatggacaagtggatttggtcaatgttctcgggagggacatcaaagactatggcttcgttgtaaacaggattcaaggtgttcctcttggtggatgttttcctcttcttcagtcgtctgccatcacacatcagcgagactttcacatagggatctgatgctcctgttatgtccattgcctttaaattccttgcttttataatggtaatggtcagcctgccagccgttggaagatagcacagggaaaacatcagctctcccagatccacgttgtcattggtgacatattcgatatccttccaaaggatgcactccctggggaaatcagccaagtctaggaagtgatccaccaccacttggccgattaagtcatgacgagagaacctgtcaaagtcgtacacagagaagtgaagcttccgtgcttcaaggtcattgtagggaaccggaaataaaaacacttcatcaaacacagggttcagggtctttctgtgaactttagtctggtgttttgttttccgatcaggaagcaaatagatcttgacataaggatctgaagtcccagaaaagtccttggcgggcaaattgacagctttgtgaatcttcactatgagctgctctaagtcacagtcatattttaaaatgaagttcagtttcccacaagccttgctgttactccgtctcccgtcatcattatccaatgacctctgcttatataactctggtttaattctaccaattccagtcaactgttcctgtttttgaagctgctggatattgaagtccgggtttgacaagttgagttgtcttcggattgaattatgccgggccgacgaggttggctctgtgacttggcgctgcacgcggacgccatgggcacagttctcctggatccccgtctgggtggagaggggaatgtcaggggaggtgtggctgatcttcatggaggagtcagggcagggcgtgggaggatctaggaagtcctcactgttctcctgctcattggtctctgtgtccatgtagttaaggggctcctggttgttgtctttgctaccagagggcaggcctcgttctcgccacggaacccagcagagtttccaagatacgaagagagacacgccaaagagagcgagaccacaggcagtgaccacaagggtcagcaggctcactgagatatctgggtcgcggagccggggtctggcacggtcccgcaggtggtaaatgaaatcctggcagctgtcgtgctccagggccccacgggcacagagctcggccagcagctgcagcgcctggtgacagagcgcgtccctggccccgggcatcgcccccccgcatcctcggaccgcgccgggcaggcgggcgcaggagacagccctccgcctgccagctcagagccgccgcctccgggccgtccgcgctcaccgccagggacctgccgagaaacggtgcgagcctgagcccgagccccagacccagccggcccggcctcccaccggttgcatgcagctcttcgccagccggtcggtcaggctttctc

SEQ ID NO: 10860 - RNA, 4546 nt, Homo sapiens
  source 1..4546: mol_type = other RNA
ctgaatagctgggactacaggtacattgctaattttttaaaaattagccgggggggcggggggtctcttttgaaattagatggtggtctctccatgttgccagactggtcttgaacttctggtatcaagtgatcctcccgccttggcctcccaaagtgctgagattacaggtgtgagtcactgcacccagccctaaatcataccatttagagtcatgattgttggagaattttgaaaacatctgcattgtagaaacctttcccctcccctccctgacccttgctcctgtcatgtaccagtgtacttcctggacatcaaagtgcctgctgcatatgtccaactcactggctgggagggtgcttcagcagcaacacacatcaagggcaggtctccttgaagccaacagaagtaagaggaaggggctgagaatcagtgccagttgggtggggggacacctggcctctccctctctcggcaccagcttttcccaaggtctgatcagaatgtttcctttctactgccatgtccattttttcatggtattttaatttccttctttatcctggaaaagacattggagaatccccttcccccaagttaaataagacaaggttggagtttttcaaaaggagcatttactaggaaactaaagggcaaccaaacagaatgcaagagaacagaggcagagttgcaaatgggctgagggagttcaaatttataaccagcctctgctcacagctgtactggctaggcaaagctttccagacacaaagccacctgcctgccatgtggatagtactctttgcctgcttgcccctacaaagccaccttctatttcataccaataagccagttgcatcctcattagtatcccaaggctgctggctctctgggcaggaagcttctgaggtggggaacagtaggcacagctgcctcaggatctccaacccaggcttccattgccaaggacatgtcagaatttattgggattgctgcctgatatctattggagccagtctgctttctctgggaccattcttctgggctcatctgcctagctttacagacaatatttctgctaactatcctggtggcgctagcccttcatgttttgcttctaaacactggtatggtggaggatgtctgaatgaggagggatgagcagaggggaaccttgagcagaggaagccaagttttccttatgtcatcagacataggcagaaccttggattctctttgaatcccagtggttggaagccaatcagagaagtgaagcttgaatgtaatgacactgcttcctacaaacaaaggcctatagccttcttagatctgccatcaaagtagagcttcttgtatagtactaggcagctggggcaatgagaactttctgaagacgtataacgatccttcctccgcccagttagttccatgctgaaatgttaattcaaacagagataatgagctttccaggaaggtaaactacaatccaactctggattctgctgtaaagagattgtgtgaaaagaaaaatactatcttggagtagtggtgcaaatgtgtggatggggtgccttgcacctataatgggacagagaggaccattaggtaacagcccccagtcctcccaggatatgctgaggcctttggtttcatttacgtggaggcagaagcaatgaggatgaggcgcatagctggccattggttggcagacttggtcaggaaggaagctgagtaatgaatgagatgcctggggagggcccttgaccttcactcttgtaggtatttccatccccaagtggtgtgaaagtgatgtatgtgtctgaagtgagaaggaaacctctatgtgtggttgcccaaggctatgactctgggctgttgcatatggaaataccccagaaggcattcaggccagagaagcccaaaagctgtgcctttctataggggatggctgtgttctctctccatgatctcatctcacccattgctgtaccagtttctgaggctgttcccttagtggacgaatgtgcctaggaaaggatattccacaatgctcatgccactgagatgtatgcccttctaactaattacttttcattctaataacactcccagttgaaaggaaggggctgctagctactgagtgagtagtgttgggggtctctgattcctcaaaatctggttttagcagaaaacagggccatgttgatactggtactctctaccacgtgcatgggaggaggcagtgaatttgctgtgaactagccctccttgcattagattttttccagggaacagcctgcttgtcttggtattctcttggggctattccttgcaaatctggagcacttcttggggcacagttattttctggagacagtcattagctcaaaggtagtcatgtgtgaattgagatctgctgcctatttagcacctggatatatttttaaatattctgtccttccagggcattctagaaaataatattatgttggaataacgatttccagggcagatgctatgtcctcatcaccaagggcttcatatgaaacattgagtcctggtactcttggtactgtcactatatctatcatttgtttttgttcatagtccgatcttggttcttggcatgagagacatgcttccctgcagcacatcaccttgggccacctgcagaaggtggctggaccattcaggttcaccaaacccaatctggaaagaaggccagttagtgctgtggttacagctgagcatttggtcactgaaatcgtctggatgttgctggatggaaaaagttacttaagatctttgtgagatggttgtcctattttgtccttggcacaagcagtcctcttacccatggtcatcgtttctccaccagggaatgccagtgtgcaatgggcttccgaggatatgacaacatttcactccagtggtctctgcccagcctctcagcctcgttgcctacttgacacacgccgatgatctcattgtgaccggtcatagtccatgactgctatggacaagtggatttggtcaatgttctcgggagggacatcaaagactatggcttcgttgtaaacaggattcaaggtgttcctcttggtggatgttttcctcttcttcagtcgtctgccatcacacatcagcgagactttcacatagggatctgatgctcctgttatgtccattgcctttaaattccttgcttttataatggtaatggtcagcctgccagccgttggaagatagcacagggaaaacatcagctctcccagatccacgttgtcattggtgacatattcgatatccttccaaaggatgcactccctggggaaatcagccaagtctaggaagtgatccaccaccacttggccgattaagtcatgacgagagaacctgtcaaagtcgtacacagagaagtgaagcttccgtgcttcaaggtcattgtagggaaccggaaataaaaacacttcatcaaacacagggttcagggtctttctgtgaactttagtctggtgttttgttttccgatcaggaagcaaatagatcttgacataaggatctgaagtcccagaaaagtccttggcgggcaaattgacagctttgtgaatcttcactatgagctgctctaagtcacagtcatattttaaaatgaagttcagtttcccacaagccttgctgttactccgtctcccgtcatcattatccaatgacctctgcttatataactctggtttaattctaccaattccagtcaactgttcctgtttttgaagctgctggatattgaagtccgggtttgacaagttgagttgtcttcggattgaattatgccgggccgacgaggttggctctgtgacttggcgctgcacgcggacgccatgggcacagttctcctggatccccgtctgggtggagaggggaatgtcaggggaggtgtggctgatcttcatggaggagtcagggcagggcgtgggaggatctaggaagtcctcactgttctcctgctcattggtctctgtgtccatgtagttaaggggctcctggttgttgtctttgctaccagagggcaggcctcgttctcgccacggaacccagcagagtttccaagatacgaagagagacacgccaaagagagcgagaccacaggcagtgaccacaagggtcagcaggctcactgagatatctgggtcgcggagccggggtctggcacggtcccgcaggtggtaaatgaaatcctggcagctgtcgtgctccagggccccacgggcacagagctcggccagcagctgcagcgcctggtgacagagcgcgtccctggccccgggcatcgcccccccgcatcctcggaccgcgccgggcaggcgggcgcaggagacagccctccgcctgccagctcagagccgccgcctccgggccgtccgcgctcaccgccagggacctgccgagaaacggtgcgagcctgagcccgagccccagacccagccggcccggcctcccaccggttgcatgcagctcttcgccagccggtcggtcaggctttctc

SEQ ID NO: 10861 - RNA, 3041 nt, Homo sapiens
  source 1..3041: mol_type = other RNA
ctgaatagctgggactacaggtacccacaaccacacctggctaatttttgtatttttagtggaactaaaaattttattatagtattttagtttcgccattttgaccaggctggtctcaaactcctgacctcaagtgatctgccctcctcagcctcccaaagtgctgggattataggcgtgagccattgcgcccagccagtgttgttttatggaaatgagtccgtattatgcatattgctctgcagcttgttgtgttttttttccccagcttgtttttaactaacagagtatcaaatggacttccttgcaaatctgtcccattcttttaacaccaggatcacaactcaaatgcctacaggggttaggcagataacataaatgagttaaatggatccagtaggaactgcagaaaactggagatgttccatccaatggcatcagatgttacccaaccacaaactaactactgccatttggaaatgttggcccagagttgccaaatttgagttttcaagaaaagcaagaaatctgaatttttgaaatgtgcaatctccagatttttaaatattggtaacaaattcacattaaatgcagtgaaccagcccaaatgccttcaatccagacactgcccctccagccatccttttgaaacttctattgccatgtataatgttccacggtgtaactgtcaatacttaacctttctcctattgctggacacttaggctatgacattacaactactacactgaacactctgtataaatctttttgcttgtacaaataattctagaaatacagcttccaaattgccctctaaaaggctgtaccaatttatagtcctataaacactacatgagactatccttttctgggaagctttaaacagattcccaggtagtaaccctgagatcagatgcagtaggactgagatgaaacccaagactgtgtgagtgagtgatcggaatcactctcaggtgattctgatgatcagcgaggttttggaactactgttttagactatgaacaaactttggggccaggagcagtgaattgtaaaggaaactatactttcatttgtacttgttatttttttagagacagagtcttgctctatcatccaggcaggagtgcagtggtacaatgatagctcactgaagccttgaactcatgggctcaagtgatcctcccacctcagcctccagcatagcgaggccacaggcatgtgccaccatgtctggctaattttttaaaatatttttttgtagagacaggatcttgctatgttgccaggctaatctcaaactccaggcctcaaacaagcctcaaacaagcctcccacctcagcctcccaaagtccaggattacaagtgggagccactgcatctggccagtactaccatgttgtacacttttcccgctaactacagccctctatgcaaacacaaaaaaggctctgctgctgctgtttcaagcagttctgtcagagtaggacaataaataaaccaactatggaaccttcaagtggcttttattggtagagcctagaaaaagtgtcatagccatttctgagcaaaaatctgtatcccagtaaggtattcagtgttatgtttaacacactactgaaccagaaagtttaagttcctgacacagacgcaaccaggtcactaagaggctccaaaatcaacaagttaagccctgctgctctgttaagatctgaaaggcaagacacagtcctggatgtgtgcccttgttacggggtgactaaaaaggcaggcaacagtatcaaggattttttttttaggtggactcctgtgcactcccacattgcaaggatgtgcttcagcagcaacactcaagtctcctcttcattctgtatctgcctaagcaatctgcttaggacacgtgtggtcggtcataaaacatgatcatcaggatggtagagttcactcatcaggcggtagatgtaggaaggtgcattcccaccaatgttggagataaagagggtaatgagctctgggggaacgtagtcaaacacagggcaatgcacgctgaccttctccagaatgtccccttctgtgaatggcaggacttcttcaggagccacaaacttatgaaatgagtcttcttcattggggaactgtggagaaagtttgaacataggtgcacagacgatgagtggggtggaatggtgttttgctgccagtgccagagtgtgagttcctgtcacagctctcagggccccattggccaggatggtcttcgtgccaatgatcaccttgttgactcttgacataacggcaaaaatggcagcatcagtcatgacagttgtctcaatacctgctttggacaaattcacagccatttcatgaccctggcagaaaggagcacactctgctacaatgacatggaatttcctctttcgggcagcctctttgaggaaggcctctactgttcgggagaagccaatggtcatgatcacctcattggagtgaatgtgctccagagcctgggctgcaatgttctccattgtcccttccagctccactagcagctcattaatcgcctcaatgatgttggactggagttgggcataatggaagctgaaatcctcgtttaggcctccggatgtcaacagtttgtgcagggactcctgctgatcactctcgtcgctgcgtccatggagtctgccatactcctcccggataatcttgagcactctccgcaccatgttgcccacggtggtctcggagggctgagcggccgtcatcctcctgccctctctgcggatcagctccatcagctcccccgcgttgctccagcggtggtccgtgatgatctggcgcagcaaccctagggtctcccgagccatttcctcggagctgcgcggcccaccaccccgcttcagggtctccacgaagctctcgatcctctctgacaactccgagcccttcgctgcggatcccggcatctttaaggtagctgccttcagccttcaccggcggaatccacacctgccagaccacacagtttgcacttcc

SEQ ID NO: 10862 - RNA, 8728 nt, Homo sapiens
  source 1..8728: mol_type = other RNA
ctgaatagctgggactacaggtacccaccaccacgcccagctaatttttgtatttctagtagagacggggttccaacatgttggccaggctgctcttgaactcctgacctcaggtgatccacccgcctcggcctcccaaagtgctgggattacaggcgtgagccaccaagcccggcctgagaattctcttctgtcaatggtgtgggcctctcgacctcactaacctatattggcccagaggtgatggtgacaatttgagataacacaaagtctcaactatttacgaacctggtcatccagagagggccccggaattgctcaaatgaacagtaagaatcctgaggcagggtactgaccttggtaggtgaaataccgcctatactctcaagttttatggatagtgcagccaaattccactcggatgcctcacaactacttaaaattggctttttgaagcagcatttccctaactactcccaggaacaaagttctgtgaaatgttcatagagcttcattgaaaaaaaaaaaaaaaaaaaagctacaatatttttcttctaagatttattttataaacatgtaagaaaagttgtagatatttattgtgggtctggttatgcaagaacaatcttcctggacacagtgtgcgattctcagtatcaaaagcattctcttctttcagttcgtaaaagaaaaacatggtttaacttctaatttactgcttattataaggtttaaaagcaattactgtacttatgtatcgaacttatttgtgtagcaactaattcatctgtgaagccatggtttgctgtggcttcacagtaaattttgacttaagtctaaagcgtgtgttagcatctcaccgtaacttaatgcttcgagtgagaagtttgaggaatgctgctttaggcaaaagagccactggaggaatgagctctgctcttttcacctgctctggactgctctcactttcctcaccgacaggaccacaggcttaagaactggctcagcagtccttctttagggtctagcgcctgcctaccagcttcctctacttctatcccgggacagatgaatgcttttctaaaaaatattttggaccatctgcatgattccctagcaaatgctttagagagctggtaagcttcagctccgacatggccagatcatcaaaatttgaagtttactcaggtctatttaatgagatttttttttcttatacaaccatatgcacttctgaataatcttccctttttcgaatctggggctttcatctggaattagactaacctgcagacagtgatgccagaactgggctgggttaccataattcattcatttaccaaacactttcgaagcactacttactctgggctggcctgatgaaaggatacagagataacaccacaaagaaacttgctcattaggagcttgcttactggctagaaaggaaaatacaacatgaaaataaagcattgtacgtacatggcagaaaaatgactagcctgccagagggccccagagcctcagaggatggagccactcctgaggctggagggtttacaaactcatcccatctttacagaagacctgctagatgccaggcatgctggcaggcacaggggaaagcccactcaacaagcagacacggtccctgctctcacggagcttacagtctagcaagacaaactaggaacaagaaattacagtccagtgtagaggtgtgcagggttgtggggtacagtgatttggcattatacacacatttcgcttaaacacaatggtatttgtctgaaaaagatttaaaaaaagaaaaacaaatcagttgtttgggccattccgctggcccctccttcactccatgagcatagacaagagggcgggcccgggcaagctcatgcctctgctgcacctgcggcctgcctcagttcccaagctccccaaaagtgatcttctcgcctaaatgtggttctaacaccccaaaacaagtgatttttgcacaacacagccctaactgcaggccaatcacttcacctggtactcaaccaaacagtaatgtgttcccacatgggcaagaaatgactacatgggacctcaagatgttggtcttcaatagggcaccttccttagatttctaagaggaattttaattacactccatttttatcttaggcactgaccttagaactgaatcctggagagagctgagactcttctgtggcagtaccatgggacacatagaagtagcctataccctggctctggaagttggggactgcctcctagaagggcccctaagaccttaagttggtgaggggaagattgaggcgggagggggagaagcctgggcggaagcatgtcactggaggtagaaacagctctgtgcacagtctgtagggctagtgagatcaagatacatttagggaactggtgagcagagggcaggggagatggggagaacaggccagggatactgccagaggatagaccttggtgagcctcataacatgctatcaaaaagggtggaatttatgtatgtatgtattttttgagacaggtcttgctctgctgcccaggctggagtgcagtggcttgatcatagctcaccacagccttgaattactgggctcatgcgatcaggagtgtggaatttattctcggggcaatagtgaagctttggaaaacgttcaagcagaggaataacagaatcagatatatatttaagaaagttcatcctgaagcatgtgaaaaggtgcccgacatcattagtcattagggaaatacaaatcaaaaccacaatgagagccaggcgtggtggctcatgcctgtaatctcggcactttgggaggtcaaggcaggaggatcacttgaggccaggagtgctagacggcctgggcaacataacgaaaccccatctgtacaaaatgtattttaaaaagaaaaaataaaaacaaaaaactacaatgagataccacttcacaccagaaaataatgagtgttggtggagatgtggagaaactggaaccctcgcacactgctggtggaatggaaaatgatacagctgcttggaaaaaccacctggtggttcctgaaaaggttaaagataattatgactcagcaattccactcctaggtatatacccaagagtcatgaaaatacctgtccctgcaaaaacttgttcgggaatgttcgtagcaacactattcataatagccaaaaagtagggccaggtgcagtggctcacacctgtaatcccagaactttgggaggaagaggtgggcagatcacctgaggtcaggagttcgagaccagcctgaccaacatggtgaaaccctgtctctactaaaaatacaaaaaattagccagcgtggtggcacatgcctgtaatcccagctactctggaggctgaggcaggagaatcgcttgaaccccggaggtggaggttgcagtgggccgagatcgtgccattgcactccagcctgcacaacaagagcgaaactgtgtctcaaaaataaataatagaaatagaaatatatatatatagccctaaagtagaaacaactcaaatgcccattaaccaatgtggattaaaaaaaaggtggcatacccataaaatggactattatttggcaattttaaaaaatgaaatactgatagaagctatgacatggatgaacctcagaaatatgttaagaagccagtcacaaatagacacatagtatatgatcccatttatatgaactatccagaacaggcaaatccacagagagagaaggaagatcagtggtggccagaggctaagagggaagagggaatagggagaattgctaatggactcagggtttctttgggtgatcaaagtgttttaaaattgattacggtgctggtgcataactgtaaatatactaaaagccactcaagtgtacactttaaatggctgaactgtatgcaaattacatctaaattaagctggtaacaacaacaaaggttcatcccgctgcagtgtgcagaatggagacagggcagagaccagtgaagaggctgctgtacaaatgcagctggaaagggcagtggctgaagaacggagaggggttcacaggatcagactacaagggggccagaggaggagactacatcctgaggacgccacaaattatcctgggtacctggtaactctccagagaggagagtgggaaacaaatgaggtatctgcaattatcatcaagcagcaaacatgtatgtaaaatctcctacacataagactaagaggaacacacaaagtgtgcagccctgtgcccacatgtgtggggagtgtccagggtaaaatcacgcccagctgcctgccacgggcctgtcctgactatccattcttactcttaaactccaaagaaaaggcctcatcattcaggacacactcaagatgttgcaagatctgagtgactgagagtgggcaggagggttagagaaactaataaggccagtaactccgagaagtaaaaatctttaaagctgcctttctgggttctctctgtgtgtctgtgaaaactgtaaggttactcgagtgtgtatttctcttggttacatcaaagacccagttttgactgcacaccacctccttccagaatggcttcgctgatctgtagcaggagactgctgagtgctgaaaggccgtggaacaaatggacctgagctgctggtgtaaaaccaaaaggaaagtctgtgaaggagcatattctaaaccctgcagaggcatgccagctgggacgctgaccacaagacatctttgccccgtcagtagaagcagagactgtgctgggatgggaataagcccctgtctacacctcatgcgcgccctcagttgtctccctggcgcctcctccacctgcagtagaaattcatgctggcgagcccactgccgtcacagcttgggaagagtaaaccgccactgagatgcaccaacaaagccaggaattctggtaacagcccactcaactgctagacgggaaaactgaggcccaggtccatggagcagagccaggggttggcatccaggtgtccgattctcaggcccccgcactcctcactctaccaactccccaaaccctgacccttcctaagaacctggctctcagctgtatgcttcacagggaaagaaaagctgagaaatctcagatgtcttaagtctcaactggcagagaaaccagaaccatctctttcctagaatcctaataagaagctgaaatatatcatggttatatcctctaatctctctaaagggagggagaaaaagcaaggttaatcaacaaaatatgggacaatacagtttttgttgcagctctcaaatcttgcagccctttacttcctttattaataacagtgttctgcattaattcgtgccacagtgtaatcaactatcaatgtgaccattagctccgccacaagtaaagatcgacaggatccaggctgcactgtgtgcacaacagcccaggcaggtgaagagtcgtgacatcgcaaaaaggaccacggtttattaccatctctaacgcccatgttccagcaaaccgaagaaaaacactgtttcttaaaactgcagaggaatacaaaattaaatactacaaaacaaaaatcagacaggaagacgaaacaatctacctcctcctaatggtaaaataatctgaaaggagtttaaaaataaatgaactaaaatttttataactattatcttttctgccaattttgaagatgtcttcaggtgccacaacgtggggacagaaagaataaatatcaatgtataacttctagagtgataataaacaacaggaccccatctcagatggatggattttttttcctactggagccaaaaaacaagctgaactctatgtacaacagacagactatacaactaggagcatttaaaaataataagactcctctctctgccttcttccaaagaatagaatatatatttaacagcacaaaagacgacaccacttgagcttcccctttagccaacaggaagaatttccacatataaaaattaaaaatttaaactttcaaatcattcatgttttaaacataatacagacttaaaaattcttcaacattgacccataatcccaccccagcacaaaaatcaaccccaaatccagacgtcacagttttttgttcctaaaaatcccacagcactgaacttgatcttcacatcaagctgacagcacgtaagaggcccatgccatgagcaatccccgagggaagaacggaagcacagtcaatgctgcagctcttatctacctgggcggcactggtgcacctctgaggtcaggtccgtgagattcgccccacactagggtcccggaagggtgagctggccgcttccctcctcttccccctcgaaggatgtccaataagcacctgggaattgacttttcttgggaaaagggtgctggtaacagctgtcagggccaaggcaatagtgagaagttcagttctctgctctttggatgaactgtgtaaaacatttcttttaaaagacacaatgttaaaaatattaagaaaaatgtctacaaaatctggagggctgcctttttctcaaagggtaaagcctgtggggtggtgggaaaggaatcgagggcccagaactacaactctgcagcgaaagatagagatgcccttgaaaatgtgtcacattcttaagatgtcttgccgaagtagcaagagcggagggtgactgtgtgagcaggagcgagagggcgccagctcctgcgggggaggttcctactgcgcgccccaccctgtgcaagaatgtcaggctttagggcagctgccataggccccaggggcatcaggactctgcctctgaaccagagctgctttcccgactaacttcaatctggagagatggtaagttatctaaccggctcttcttttggcgagactgctctttctccttaatcagagccccccatgccctttgcagctcagagtcgtcttcctcagcgccaggcgccctgtgatccactttcttcgtattcttttctttggtcttgggtgcagatcctaggcgagtccataaattacctgatttcttctcccgagtatcggcgtagaggcctttactatcctgcctgggaacacctagcctactatgcacatcagaagagggctctctccgaacgacggggttactactaaaagccttttccggagaatgtggtctttttcctaaccgctggcgtatatctgatttagtactgctgactggtggccgtggacgggagtgctgacgtttctcatctaatagatgtcggacatctgcaaatttctcaggtggtaatttgttaccaattcggtttttgatattgcttgaagatacactatctgccctcatggagttcctaatatttttcaactgagattccacttcgtcagcatacatagtcattttcatgcttttctttggtgaaggcgtggaaatcattttcagttctagatcatagtccatttcatctgagtctgagctgctggcactggatcgtctagacgcgctccgctcccggggctgcttgagagccgggagctcctcgtggtactctaccaccactctgtcatctgcatccatgtcctggtcttcttcttcctcttcctcttcctcctcctcctcctcttcctcctcttcaatgggttcctcgggaacattcactagcccagaatgtcgatgtttatacgacgtcaagccaacgtcatccccaatcagggctctcttcttgatcacgtcccgctgaatacgacgggaatgatatcttcgcttccatgaattgctaagaattcctttcatgcctccataatttggattcccatatttcatgtaatactgacttcttctggctgctccaagttcctttttgtcatcttttgtagcaaatctcatgaataacctatttcctttagcaagtttgttagctggacgaagatcgtttcttaacaaagactcctcttctacctgagacaacgtatccaactctacatcacttgagttctcatcttcaacctctccttcttcagcttcatcatcatctgaactgtcttcctgcttgtcttttttccttttctcagctgacttgtcctcactggcatccctgcttctgatcttatcctgtgcaggcagggagctcatattgataagtgctcgtgtggctgtcatttcatccagccaaactacattacaggaggtatcatccaaccattcgatgtgagctggaggatattctttaaaataggaaaagacatcttgggtgctcatctcatctactccgcaaatatagattgtctccagtctcaccttggggattgctttcttcatcatgtctcggtccaaggctacatttctttgggcaagatttacttccgatcgaaaatggaagcgcttggctcgctgctctttcttttcaattgcttccttggaggtgacatcaattccagtgatgaagctgccagccttgttttcatatcttctgctcgtgtccgggatcagttccttgagcgagcgccgcacaggcacgatttccagctcgccctcctccacctccatgggctccggctcgccacggtcaacaccggactccgcctcaggggacgggagccccagggccggccccgccggggcctccgccttcaccgacacccgcaggccccgtacggccgccatcgctgcctgccggccgcaccact

SEQ ID NO: 10863 - RNA, 7296 nt, Homo sapiens
  source 1..7296: mol_type = other RNA
ctgaatagctgggactacaggtacccaccaccacgcccagctaatttttttttttcgtatttttagtagagatggggtttcactgtgttagccacgttggtctcgatctcctgaccttgtgatccgcccgcctcagcctcccaaagtgctgggattacaggcgtgagccactgcgcccggccctaatttttgtatttttagtagagttgaggtttcaccatgttggtcaggctggtctcaaacccctgacctcaagtgatccaccccgcccccgcttcggcctcccaaagcactgggattacagggatgagccacctcgctgggaccagaccttactttcttgacttggccacaagtctgtcctgctcagagctgctgaaagtggctctcctgttgtatgggcttgggtgtggtgtggtggccctttccctgtcccagctgccttcttcctgggcactgaaaacgatgctaccattgtttttttttttttttttgagacggagtctcgctctgtcgcccaggctggagtgcagtggcgggatctcggctcactgcaagctccgcctcccgggttcacaccattctcctgcctcagcctcccaagtagctgggactacaggcgcccgccactacgcccggctaattttttgtatttttagtagagacggggtttcaccgttttagccgggatggtcttgatctcctgacctcgtgatccgcccgcctcggcctcccaaagtgctgggattacaggcgtgagccaccgcgcccggccaaatgctaccattgttaagtgccaggcgtcccaccatgcgggtcttcactgcgtatccacgtagctgcaccacgcaggcattctttcctcccttttgcagatgatggcaccaaagttcaagactcgcccagggccaccaagacagtcctctagactttggtcttccctccttgcctcctcggcctggggtggtggcgcctcggtctgagaagggtcgaggtctgggtgctgctagtggccctggctcagtctcagagctgcccggagggggtgaggatggctaacttaaggagcacaggcagaggcttcctgctggcaggaagagggctgagctgcggaaggccacccaggtggagtgtgctgcacctccttcagtggccttcaggagctctgtcctcacccagggattggggtgagtcagggcatggggaaacaggctcacagagcccacctgctcaccctgaccaccccaccccaggggaccccaggctcctaactctcagaatcccacagtctgtattggcggaagacgggctggcacccttgagttaggcccccagtcgttggcacagataaggggagctgctgctgaaggagcccgacggctgattctgtggaggcttctcagagctcctggcaggagcccctcaccgcaggaggcccacaacccctcccagctgcatatcggctcacattcacgcggctgccacacaagtgcgtcggaaactccacttggctgaacgtgattgtgctgctgtctgggacagtcttatgcacgtgagcccaatactggatgtcccgccattttcagccctggggcctatggcaaagtgacgcccccctcggagtgcacggcaggcaaggaaggtttaaacggaagttctgaccaggacgatgctgggtgcaagaggggacggggatggagcaaaacagaaaggatccaccagggcctgcaaccacgtctttggccccggtgaggggtgggaccttgtgtataggtccaggcagcagcagctgcagacagaggcctagagggtttggagaaggccgaccacaaagacacgcctagaccccagagtctagtgaggagagggactgggggcagtgtttcggcagcagacccagacccagactcagacccaagcccccctcctcactgatcaaaaccccaagggcagggagcccttcctgctccttcccgccagagcctggaggatgaggggcagacgggaggcccggccactggtgcctgctcctttgatcagctgtagtcccttccccttcacagggcacttgtcttgctggttggggtcaccagggattgctcccccaagtacccatcagcctccagggcccaaatgattccatgcagtagctctctccccctcttctgagaaggctcttggctcccagaaacggaaaccatgcctgggcctgctccccttccttgggctgtgacccccctgccacagaggccccccccccgccacagaggtcccccctgccacagaggtccccctgccacagaggcctggtggcccctgagctgctgctccgagtggaatgtcctggtctagaggcccttggctgctccagtgtcttaagacccatatatgagtgctggctctgaccttgaacaagctcctccatcgctccaggcctcgtttttcaggtgtatatgatgatagtatctctaggcctcgtttttcagttgtaaagcagggatgatcatatgtgtttaactcccagattgttatcaagtcaaggacaacaataggaaaacatgtcacctgtcagctccacacaaggcaaagtaggatgggtgacccctgactagggggtgggagtgcagggggcacccgacccatctggccagccacagcctctgtaccctgctcgcattttcaggcctcaatccccaagcactgttggccctggactgtttccccccctcaattctgtttctcaatgcctgcttcttcccagtaagtgccacaccctgagggtgggtgggagagtgaggcagcactgcccactttggctgggactgggcactgctggggacagcacgggccacgtcttccccatctcaagactggctttttggctaggcattgtgactcacgcctgtaatctcagcactttgggaggctgaggtgggagaattgcttcagcccaggagttccagaccagcctgggcaaaatagcaagaattcatctttatgaaaaagaaaaaaaaaattagccaggcatggtggcacacacttatagtcccagatacttaggaggccgaggtgggaggatcccttgagcccatgagttggaggccgtggtgagctatcagttgcaccactgcactccagcctggatggcagagcaagaccccaactcaaaaaaaaaaaaaaaaaaaaaaaggcggccttttcccagctggcagcaccctggctagttagggtttctccgaatctgcaactcctgtgtgatggcgggtctcaaatgctggcagcagagtcaccggtcagcggcaagacctggagtctccatttggaaccagcacccgggagcctctgctgggggtgatcatggagccgcacgtggaggctggtggctctgatggttcgagccgttcctcggcagcacagcacacccgctcctgaggagccacggagctcatgagcgttggcaaagtgctgtcagtgctggctgtaaggaaacaggcttgacttttaactcagcctttcccaaacttgactataatactttcttgaaaatcagaataaccactaacatcacaaaacgagtgttctcaggagtgggcatgtttatctcgttctctttttttttttctttttgagacggagcctcgctctgttgcccaggctggagtgcaatggtgcgatctcgactcacggcaatctccgtctccccggttcaagcgattctcctgcctcaggctcccgagtagttgggattacaggcgcacgccaccacgcccgattaatgtttatttttagtacagacggggtttctccatgttggtcaggatggtctcgaactcctgacctcaggtgagcctcctgccttggcctcccaaagtgctgggattataggcgtgagccaccacgcccagtctttttttaaatatttgagtgaaataaagcctaggagatatgtgttccaggcgcccaagctgttaatgtggagcttgaatgtggcctggacctgccctttcctcttctcctttcatccccctccctgccgcccacatcctgaactgctctgagcctgcagaagaacccagcgggaatcttcagggttgtggaagggtgtagggatggaaagggaccaggattcgcctgtttggctgggaaaatcggtagaggagggtggctcacacttctaagatgtctgcacaagcccagtttgtttgggggttggggaggaaggtcttttcctggcccactgtccctcccgagtcagcagtcccccagagagacgaagagcagctgggcacggctggagctggtcggtggcagagaatcttgtcctgccttttcttctcaagctcaaaataggcacatgcagctattaactgatatgccagaaggggcatcccttacccggaggaaaatggatttattgctttataaaaaagaagtctaataaaactgaagagaaaataactaaaaatccaaacacaactcacccctctaagcacgcccaggaggtctcaagacacacttctgggggcagtcaaggtgggcgggttggtgggccaggcggacgggcctcccccgtcatcagctccagggccccacggagcccgccggcagggggtgctgtgggcctgtggccttggacaagctcctggccccacgccaggatggctcctgggcactggcccagctgcaggcctggcggctcccgcctggtcagtggggataagggctaactcctagagcccaccccgaccccacacacacctcggacccacccacgtccccaccccggcctggacctccacgtctgccggccacagcctttcgtccacctccacaaaagcagctgtgtgtatgtacggggtgccctggcggcggtcctcaaattcccttcaggtggcagacagaacgagggtgacagtgaaaacgtgtccgcggcattggccctcggggaggaggcgaggggtccacccagcccgctaaaccctctccagggcataagccaggtggggcttctccaccggcctccaacgggtgggcaggccctggacaggcgacagggggctggaattacaaaggaattagcaccgacaacaggaagcgggtccttccttcctcaggcagcctcaggctggccggggagggggtgggggccaggcgcgggcgagacagtgcaagcctttgtcctcaggcaggtacggctgtgggcatgcagccgaggggcaggtggcaggcaggggatggcagccccctctgctttggcaagaggcagaatccagacactggcgggagagcgcctgcctgccgggcgttcctggctcctgctgcaggcaccacagagaccccaggccccgggtccccggggggcggcagagcaaagtcagggcagcccctgcgttcggcaggagaaaacgcgcgtgtccggggccctctcccgtccttccaccacagagctccgaggcagggccccgggagggagcgtgaacgctggcacggagacggcgaaggtcctgggggtgcgtggggtactctggaggggcaggacaggggtcagtcactgaagcacaggcaggagaccgcagttccgaggcggcagccactacacgaaggcctcctggttggacgagccgttgattttgaggaagagtttgtcatcctcctgcctctgctgcagctgccgctccagctggcgccggtagcagatcaggtagagcgggaggcagaagcccagcaggctgagaaggagcagccccacgttcacccacagagggtctccctggagaggacccatcatggccagaaacagcggctgctgcagaagggcgaagagcgcgctgatcagagactgcagtcccgtgaggctgccgaactgggtggaggggtacacggcagcgtacaggcccccgacagcggagtggatgaatcctcgcacgattgtgtgcaggatgaaggagaggatctggagaggcaggttgggaatgaggcaggtcaccccaaagcccacgagcagcaggttggtgaaggcgaaggcccgcatggcattagtgatcttctggatctgccggtcccgcttcttctttttcttctcgcctctgtcttctggtcgccgctgaccaggaacttgaggatgttgttcatagcccccatgtagaagatgagccgcagctgcgtgacgcacatggtgaccaggctgagcagcaggatggggctgaacacgctgtgcatgaaggagggggccactgcggcatccggctggcacttcacctccaggtcgacggtggacaggcacagcttgtggccctcctgcagcgccacctgctccttggcactcctcatggagctgcccacactcaggcgccggcccaccgtggtcacctgcttgtagaactgcttccctgtgatcttgtggtcaaagcccagccagctgaacttgatcttcaccgagtagtccatgtcctccggccccgggaagggctcaaggggccagttaaagaagcagttgaggaaaaccagcccggagcagccggcccagaccacgaggacgacgatgaaggagacaccagcatcatagatgagcttgattcctggaaaggtgactgccgaggaggcgtaggacccaatcatcaaggcaataaacgtggaccgaaggtcgccgaacatgttgggcagtgttaatgaggtgaaggtcatacacatcccaccaaagccattcagagccagggcgatgaagatgagcacggagagagcgtttggtttacttgctccgtacgcaatcagcaagcaggaaaccgcgaagcaggcgctgcccagcagcctgagcttcctcgggccatacttgtccatgacgatacccaggggcagggtgatggcactgagcagaaaggagcccacagtgaaggccaaatttagcatctcgtcctgggcctggcagctgagccagccgttcatccagctcacctcctcgtgccccggctctgctgtgccgcccactgtgccattggtgacattctctggctcggtacacaggtaggagtaaaagccctctgacttgagcatgatgagcagcgagccccagcccaggaggactgccgagaagaggaggttctccagcacggccgtgcaggccatccaccagcggcgccgatgggcagtggccagggtgggcgccatggtgcggcgcggcgcggctccggctccggctccggctctgcaccacccggctcctccggcgtgtgtcgggcccgcccggcgccttttctgccctcttttattccagcccttttattccgaccccaagaagaa

SEQ ID NO: 10864 - RNA, 7402 nt, Homo sapiens
  source 1..7402: mol_type = other RNA
ctgaatagctgggactacaggtacccaccaccacgcccagctaatttttttttttcgtatttttagtagagatggggtttcactgtgttagccacgttggtctcgatctcctgaccttgtgatccgcccgcctcagcctcccaaagtgctgggattacaggcgtgagccactgcgcccggccctaatttttgtatttttagtagagttgaggtttcaccatgttggtcaggctggtctcaaacccctgacctcaagtgatccaccccgcccccgcttcggcctcccaaagcactgggattacagggatgagccacctcgctgggaccagaccttactttcttgacttggccacaagtctgtcctgctcagagctgctgaaagtggctctcctgttgtatgggcttgggtgtggtgtggtggccctttccctgtcccagctgccttcttcctgggcactgaaaacgatgctaccattgtttttttttttttttttgagacggagtctcgctctgtcgcccaggctggagtgcagtggcgggatctcggctcactgcaagctccgcctcccgggttcacaccattctcctgcctcagcctcccaagtagctgggactacaggcgcccgccactacgcccggctaattttttgtatttttagtagagacggggtttcaccgttttagccgggatggtcttgatctcctgacctcgtgatccgcccgcctcggcctcccaaagtgctgggattacaggcgtgagccaccgcgcccggccaaatgctaccattgttaagtgccaggcgtcccaccatgcgggtcttcactgcgtatccacgtagctgcaccacgcaggcattctttcctcccttttgcagatgatggcaccaaagttcaagactcgcccagggccaccaagacagtcctctagactttggtcttccctccttgcctcctcggcctggggtggtggcgcctcggtctgagaagggtcgaggtctgggtgctgctagtggccctggctcagtctcagagctgcccggagggggtgaggatggctaacttaaggagcacaggcagaggcttcctgctggcaggaagagggctgagctgcggaaggccacccaggtggagtgtgctgcacctccttcagtggccttcaggagctctgtcctcacccagggattggggtgagtcagggcatggggaaacaggctcacagagcccacctgctcaccctgaccaccccaccccaggggaccccaggctcctaactctcagaatcccacagtctgtattggcggaagacgggctggcacccttgagttaggcccccagtcgttggcacagataaggggagctgctgctgaaggagcccgacggctgattctgtggaggcttctcagagctcctggcaggagcccctcaccgcaggaggcccacaacccctcccagctgcatatcggctcacattcacgcggctgccacacaagtgcgtcggaaactccacttggctgaacgtgattgtgctgctgtctgggacagtcttatgcacgtgagcccaatactggatgtcccgccattttcagccctggggcctatggcaaagtgacgcccccctcggagtgcacggcaggcaaggaaggtttaaacggaagttctgaccaggacgatgctgggtgcaagaggggacggggatggagcaaaacagaaaggatccaccagggcctgcaaccacgtctttggccccggtgaggggtgggaccttgtgtataggtccaggcagcagcagctgcagacagaggcctagagggtttggagaaggccgaccacaaagacacgcctagaccccagagtctagtgaggagagggactgggggcagtgtttcggcagcagacccagacccagactcagacccaagcccccctcctcactgatcaaaaccccaagggcagggagcccttcctgctccttcccgccagagcctggaggatgaggggcagacgggaggcccggccactggtgcctgctcctttgatcagctgtagtcccttccccttcacagggcacttgtcttgctggttggggtcaccagggattgctcccccaagtacccatcagcctccagggcccaaatgattccatgcagtagctctctccccctcttctgagaaggctcttggctcccagaaacggaaaccatgcctgggcctgctccccttccttgggctgtgacccccctgccacagaggccccccccccgccacagaggtcccccctgccacagaggtccccctgccacagaggcctggtggcccctgagctgctgctccgagtggaatgtcctggtctagaggcccttggctgctccagtgtcttaagacccatatatgagtgctggctctgaccttgaacaagctcctccatcgctccaggcctcgtttttcaggtgtatatgatgatagtatctctaggcctcgtttttcagttgtaaagcagggatgatcatatgtgtttaactcccagattgttatcaagtcaaggacaacaataggaaaacatgtcacctgtcagctccacacaaggcaaagtaggatgggtgacccctgactagggggtgggagtgcagggggcacccgacccatctggccagccacagcctctgtaccctgctcgcattttcaggcctcaatccccaagcactgttggccctggactgtttccccccctcaattctgtttctcaatgcctgcttcttcccagtaagtgccacaccctgagggtgggtgggagagtgaggcagcactgcccactttggctgggactgggcactgctggggacagcacgggccacgtcttccccatctcaagactggctttttggctaggcattgtgactcacgcctgtaatctcagcactttgggaggctgaggtgggagaattgcttcagcccaggagttccagaccagcctgggcaaaatagcaagaattcatctttatgaaaaagaaaaaaaaaattagccaggcatggtggcacacacttatagtcccagatacttaggaggccgaggtgggaggatcccttgagcccatgagttggaggccgtggtgagctatcagttgcaccactgcactccagcctggatggcagagcaagaccccaactcaaaaaaaaaaaaaaaaaaaaaaaggcggccttttcccagctggcagcaccctggctagttagggtttctccgaatctgcaactcctgtgtgatggcgggtctcaaatgctggcagcagagtcaccggtcagcggcaagacctggagtctccatttggaaccagcacccgggagcctctgctgggggtgatcatggagccgcacgtggaggctggtggctctgatggttcgagccgttcctcggcagcacagcacacccgctcctgaggagccacggagctcatgagcgttggcaaagtgctgtcagtgctggctgtaaggaaacaggcttgacttttaactcagcctttcccaaacttgactataatactttcttgaaaatcagaataaccactaacatcacaaaacgagtgttctcaggagtgggcatgtttatctcgttctctttttttttttctttttgagacggagcctcgctctgttgcccaggctggagtgcaatggtgcgatctcgactcacggcaatctccgtctccccggttcaagcgattctcctgcctcaggctcccgagtagttgggattacaggcgcacgccaccacgcccgattaatgtttatttttagtacagacggggtttctccatgttggtcaggatggtctcgaactcctgacctcaggtgagcctcctgccttggcctcccaaagtgctgggattataggcgtgagccaccacgcccagtctttttttaaatatttgagtgaaataaagcctaggagatatgtgttccaggcgcccaagctgttaatgtggagcttgaatgtggcctggacctgccctttcctcttctcctttcatccccctccctgccgcccacatcctgaactgctctgagcctgcagaagaacccagcgggaatcttcagggttgtggaagggtgtagggatggaaagggaccaggattcgcctgtttggctgggaaaatcggtagaggagggtggctcacacttctaagatgtctgcacaagcccagtttgtttgggggttggggaggaaggtcttttcctggcccactgtccctcccgagtcagcagtcccccagagagacgaagagcagctgggcacggctggagctggtcggtggcagagaatcttgtcctgccttttcttctcaagctcaaaataggcacatgcagctattaactgatatgccagaaggggcatcccttacccggaggaaaatggatttattgctttataaaaaagaagtctaataaaactgaagagaaaataactaaaaatccaaacacaactcacccctctaagcacgcccaggaggtctcaagacacacttctgggggcagtcaaggtgggcgggttggtgggccaggcggacgggcctcccccgtcatcagctccagggccccacggagcccgccggcagggggtgctgtgggcctgtggccttggacaagctcctggccccacgccaggatggctcctgggcactggcccagctgcaggcctggcggctcccgcctggtcagtggggataagggctaactcctagagcccaccccgaccccacacacacctcggacccacccacgtccccaccccggcctggacctccacgtctgccggccacagcctttcgtccacctccacaaaagcagctgtgtgtatgtacggggtgccctggcggcggtcctcaaattcccttcaggtggcagacagaacgagggtgacagtgaaaacgtgtccgcggcattggccctcggggaggaggcgaggggtccacccagcccgctaaaccctctccagggcataagccaggtggggcttctccaccggcctccaacgggtgggcaggccctggacaggcgacagggggctggaattacaaaggaattagcaccgacaacaggaagcgggtccttccttcctcaggcagcctcaggctggccggggagggggtgggggccaggcgcgggcgagacagtgcaagcctttgtcctcaggcaggtacggctgtgggcatgcagccgaggggcaggtggcaggcaggggatggcagccccctctgctttggcaagaggcagaatccagacactggcgggagagcgcctgcctgccgggcgttcctggctcctgctgcaggcaccacagagaccccaggccccgggtccccggggggcggcagagcaaagtcagggcagcccctgcgttcggcaggagaaaacgcgcgtgtccggggccctctcccgtccttccaccacagagctccgaggcagggccccgggagggagcgtgaacgctggcacggagacggcgaaggtcctgggggtgcgtggggtactctggaggggcaggacaggggtcagtcactgaagcacaggcaggagaccgcagttccgaggcggcagccactacacgaaggcctcctggttggacgagccgttgattttgaggaagagtttgtcatcctcctgcctctgctgcagctgccgctccagctggcgccggtagcagatcaggtagagcgggaggcagaagcccagcaggctgagaaggagcagccccacgttcacccacagagggtctccctggagaggacccatcatggccagaaacagcggctgctgcagaagggcgaagagcgcgctgatcagagactgcagtcccgtgaggctgccgaactgggtggaggggtacacggcagcgtacaggcccccgacagcggagtggatgaatcctcgcacgattgtgtgcaggatgaaggagaggatctggagaggcaggttgggaatgaggcaggtcaccccaaagcccacgagcagcaggttggtgaaggcgaaggcccgcatggcattagtgatcttctggatctgccggtcccgcttcttctttttcttctcgccttggttggcgtctttctcctcgggctcctcggaggcgtcttcacactccttcagcctccagtccatgatgtagccaatgacgggggccgtcagcaggcacagcagctggagcacgccgaagatggaggtgtagaggccaaccgtggccatcactgtcttctggtcgccgctgaccaggaacttgaggatgttgttcatagcccccatgtagaagatgagccgcagctgcgtgacgcacatggtgaccaggctgagcagcaggatggggctgaacacgctgtgcatgaaggagggggccactgcggcatccggctggcacttcacctccaggtcgacggtggacaggcacagcttgtggccctcctgcagcgccacctgctccttggcactcctcatggagctgcccacactcaggcgccggcccaccgtggtcacctgcttgtagaactgcttccctgtgatcttgtggtcaaagcccagccagctgaacttgatcttcaccgagtagtccatgtcctccggccccgggaagggctcaaggggccagttaaagaagcagttgaggaaaaccagcccggagcagccggcccagaccacgaggacgacgatgaaggagacaccagcatcatagatgagcttgattcctggaaaggtgactgccgaggaggcgtaggacccaatcatcaaggcaataaacgtggaccgaaggtcgccgaacatgttgggcagtgttaatgaggtgaaggtcatacacatcccaccaaagccattcagagccagggcgatgaagatgagcacggagagagcgtttggtttacttgctccgtacgcaatcagcaagcaggaaaccgcgaagcaggcgctgcccagcagcctgagcttcctcgggccatacttgtccatgacgatacccaggggcagggtgatggcactgagcagaaaggagcccacagtgaaggccaaatttagcatctcgtcctgggcctggcagctgagccagccgttcatccagctcacctcctcgtgccccggctctgctgtgccgcccactgtgccattggtgacattctctggctcggtacacaggtaggagtaaaagccctctgacttgagcatgatgagcagcgagccccagcccaggaggactgccgagaagaggaggttctccagcacggccgtgcaggccatccaccagcggcgccgatgggcagtggccagggtgggcgccatggtgcggcgcggcgcggctccggctccggctccggctctgcaccacccggctcctccggcgtgtgtcgggcccgcccggcgcctttt

SEQ ID NO: 10865 - RNA, 7664 nt, Homo sapiens
  source 1..7664: mol_type = other RNA
ctgaatagctgggactacaggtacccaccaccacgcccagctaatttttttttttcgtatttttagtagagatggggtttcactgtgttagccacgttggtctcgatctcctgaccttgtgatccgcccgcctcagcctcccaaagtgctgggattacaggcgtgagccactgcgcccggccctaatttttgtatttttagtagagttgaggtttcaccatgttggtcaggctggtctcaaacccctgacctcaagtgatccaccccgcccccgcttcggcctcccaaagcactgggattacagggatgagccacctcgctgggaccagaccttactttcttgacttggccacaagtctgtcctgctcagagctgctgaaagtggctctcctgttgtatgggcttgggtgtggtgtggtggccctttccctgtcccagctgccttcttcctgggcactgaaaacgatgctaccattgtttttttttttttttttgagacggagtctcgctctgtcgcccaggctggagtgcagtggcgggatctcggctcactgcaagctccgcctcccgggttcacaccattctcctgcctcagcctcccaagtagctgggactacaggcgcccgccactacgcccggctaattttttgtatttttagtagagacggggtttcaccgttttagccgggatggtcttgatctcctgacctcgtgatccgcccgcctcggcctcccaaagtgctgggattacaggcgtgagccaccgcgcccggccaaatgctaccattgttaagtgccaggcgtcccaccatgcgggtcttcactgcgtatccacgtagctgcaccacgcaggcattctttcctcccttttgcagatgatggcaccaaagttcaagactcgcccagggccaccaagacagtcctctagactttggtcttccctccttgcctcctcggcctggggtggtggcgcctcggtctgagaagggtcgaggtctgggtgctgctagtggccctggctcagtctcagagctgcccggagggggtgaggatggctaacttaaggagcacaggcagaggcttcctgctggcaggaagagggctgagctgcggaaggccacccaggtggagtgtgctgcacctccttcagtggccttcaggagctctgtcctcacccagggattggggtgagtcagggcatggggaaacaggctcacagagcccacctgctcaccctgaccaccccaccccaggggaccccaggctcctaactctcagaatcccacagtctgtattggcggaagacgggctggcacccttgagttaggcccccagtcgttggcacagataaggggagctgctgctgaaggagcccgacggctgattctgtggaggcttctcagagctcctggcaggagcccctcaccgcaggaggcccacaacccctcccagctgcatatcggctcacattcacgcggctgccacacaagtgcgtcggaaactccacttggctgaacgtgattgtgctgctgtctgggacagtcttatgcacgtgagcccaatactggatgtcccgccattttcagccctggggcctatggcaaagtgacgcccccctcggagtgcacggcaggcaaggaaggtttaaacggaagttctgaccaggacgatgctgggtgcaagaggggacggggatggagcaaaacagaaaggatccaccagggcctgcaaccacgtctttggccccggtgaggggtgggaccttgtgtataggtccaggcagcagcagctgcagacagaggcctagagggtttggagaaggccgaccacaaagacacgcctagaccccagagtctagtgaggagagggactgggggcagtgtttcggcagcagacccagacccagactcagacccaagcccccctcctcactgatcaaaaccccaagggcagggagcccttcctgctccttcccgccagagcctggaggatgaggggcagacgggaggcccggccactggtgcctgctcctttgatcagctgtagtcccttccccttcacagggcacttgtcttgctggttggggtcaccagggattgctcccccaagtacccatcagcctccagggcccaaatgattccatgcagtagctctctccccctcttctgagaaggctcttggctcccagaaacggaaaccatgcctgggcctgctccccttccttgggctgtgacccccctgccacagaggccccccccccgccacagaggtcccccctgccacagaggtccccctgccacagaggcctggtggcccctgagctgctgctccgagtggaatgtcctggtctagaggcccttggctgctccagtgtcttaagacccatatatgagtgctggctctgaccttgaacaagctcctccatcgctccaggcctcgtttttcaggtgtatatgatgatagtatctctaggcctcgtttttcagttgtaaagcagggatgatcatatgtgtttaactcccagattgttatcaagtcaaggacaacaataggaaaacatgtcacctgtcagctccacacaaggcaaagtaggatgggtgacccctgactagggggtgggagtgcagggggcacccgacccatctggccagccacagcctctgtaccctgctcgcattttcaggcctcaatccccaagcactgttggccctggactgtttccccccctcaattctgtttctcaatgcctgcttcttcccagtaagtgccacaccctgagggtgggtgggagagtgaggcagcactgcccactttggctgggactgggcactgctggggacagcacgggccacgtcttccccatctcaagactggctttttggctaggcattgtgactcacgcctgtaatctcagcactttgggaggctgaggtgggagaattgcttcagcccaggagttccagaccagcctgggcaaaatagcaagaattcatctttatgaaaaagaaaaaaaaaattagccaggcatggtggcacacacttatagtcccagatacttaggaggccgaggtgggaggatcccttgagcccatgagttggaggccgtggtgagctatcagttgcaccactgcactccagcctggatggcagagcaagaccccaactcaaaaaaaaaaaaaaaaaaaaaaaggcggccttttcccagctggcagcaccctggctagttagggtttctccgaatctgcaactcctgtgtgatggcgggtctcaaatgctggcagcagagtcaccggtcagcggcaagacctggagtctccatttggaaccagcacccgggagcctctgctgggggtgatcatggagccgcacgtggaggctggtggctctgatggttcgagccgttcctcggcagcacagcacacccgctcctgaggagccacggagctcatgagcgttggcaaagtgctgtcagtgctggctgtaaggaaacaggcttgacttttaactcagcctttcccaaacttgactataatactttcttgaaaatcagaataaccactaacatcacaaaacgagtgttctcaggagtgggcatgtttatctcgttctctttttttttttctttttgagacggagcctcgctctgttgcccaggctggagtgcaatggtgcgatctcgactcacggcaatctccgtctccccggttcaagcgattctcctgcctcaggctcccgagtagttgggattacaggcgcacgccaccacgcccgattaatgtttatttttagtacagacggggtttctccatgttggtcaggatggtctcgaactcctgacctcaggtgagcctcctgccttggcctcccaaagtgctgggattataggcgtgagccaccacgcccagtctttttttaaatatttgagtgaaataaagcctaggagatatgtgttccaggcgcccaagctgttaatgtggagcttgaatgtggcctggacctgccctttcctcttctcctttcatccccctccctgccgcccacatcctgaactgctctgagcctgcagaagaacccagcgggaatcttcagggttgtggaagggtgtagggatggaaagggaccaggattcgcctgtttggctgggaaaatcggtagaggagggtggctcacacttctaagatgtctgcacaagcccagtttgtttgggggttggggaggaaggtcttttcctggcccactgtccctcccgagtcagcagtcccccagagagacgaagagcagctgggcacggctggagctggtcggtggcagagaatcttgtcctgccttttcttctcaagctcaaaataggcacatgcagctattaactgatatgccagaaggggcatcccttacccggaggaaaatggatttattgctttataaaaaagaagtctaataaaactgaagagaaaataactaaaaatccaaacacaactcacccctctaagcacgcccaggaggtctcaagacacacttctgggggcagtcaaggtgggcgggttggtgggccaggcggacgggcctcccccgtcatcagctccagggccccacggagcccgccggcagggggtgctgtgggcctgtggccttggacaagctcctggccccacgccaggatggctcctgggcactggcccagctgcaggcctggcggctcccgcctggtcagtggggataagggctaactcctagagcccaccccgaccccacacacacctcggacccacccacgtccccaccccggcctggacctccacgtctgccggccacagcctttcgtccacctccacaaaagcagctgtgtgtatgtacggggtgccctggcggcggtcctcaaattcccttcaggtggcagacagaacgagggtgacagtgaaaacgtgtccgcggcattggccctcggggaggaggcgaggggtccacccagcccgctaaaccctctccagggcataagccaggtggggcttctccaccggcctccaacgggtgggcaggccctggacaggcgacagggggctggaattacaaaggaattagcaccgacaacaggaagcgggtccttccttcctcaggcagcctcaggctggccggggagggggtgggggccaggcgcgggcgagacagtgcaagcctttgtcctcaggcaggtacggctgtgggcatgcagccgaggggcaggtggcaggcaggggatggcagccccctctgctttggcaagaggcagaatccagacactggcgggagagcgcctgcctgccgggcgttcctggctcctgctgcaggcaccacagagaccccaggccccgggtccccggggggcggcagagcaaagtcagggcagcccctgcgttcggcaggagaaaacgcgcgtgtccggggccctctcccgtccttccaccacagagctccgaggcagggccccgggagggagcgtgaacgctggcacggagacggcgaaggtcctgggggtgcgtggggtactctggaggggcaggacaggggtcagtcactgaagcacaggcaggagaccgcagttccgaggcggcagccactacacgaaggcctcctggttggacgagccgttgattttgaggaagagtttgtcatcctcctgcctctgctgcagctgccgctccagctggcgccggtagcagatcaggtagagcgggaggcagaagcccagcaggctgagaaggagcagccccacgttcacccacagagggtctccctggagaggacccatcatggccagaaacagcggctgctgcagaagggcgaagagcgcgctgatcagagactgcagtcccgtgaggctgccgaactgggtggaggggtacacggcagcgtacaggcccccgacagcggagtggatgaatcctcgcacgattgtgtgcaggatgaaggagaggatctggagaggcaggttgggaatgaggcaggtcaccccaaagcccacgagcagcaggttggtgaaggcgaaggcccgcatggcattagtgatcttctggatctgccggtcccgcttcttctttttcttctcgccttggttggcgtctttctcctcgggctcctcggaggcgtcttcacactccttcagcctccagtccatgatgtagccaatgacgggggccgtcagcaggcacagcagctggagcacgccgaagatggaggtgtagaggccaaccgtggccatcactgtcttctggtcgccgctgaccaggaacttgaggatgttgttcatagcccccatgtagaagatgagccgcagctgcgtgacgcacatggtgaccaggctgagcagcaggatggggctgaacacgctgtgcatgaaggagggggccactgcggcatccggctggcacttcacctccaggtcgacggtggacaggcacagcttgtggccctcctgcagcgccacctgctccttggcactcctcatggagctgcccacactcaggcgccggcccaccgtggtcacctgcttgtagaactgcttccctgtgatcttgtggtcaaagcccagccagctgaacttgatcttcaccgagtagtccatgtcctccggccccgggaagggctcaaggggccagttaaagaagcagttgaggaaaaccagcccggagcagccggcccagaccacgaggacgacgatgaaggagacaccagcatcatagatgagcttgattcctggaaaggtgactgccgaggaggcgtaggacccaatcatcaaggcaataaacgtggaccgaaggtcgccgaacatgttgggcagtgttaatgaggtgaaggtcatacacatcccaccaaagccattcagagccagggcgatgaagatgagcacggagagagcgtttggtttacttgctccgtacgcaatcagcaagcaggaaaccgcgaagcaggcgctgcccagcagcctgagcttcctcgggccatacttgtccatgacgatacccaggggcagggtgatggcactgagcagaaaggagcccacagtgaaggccaaatttagcatctcgtcctgggcctggcagctgagccagccgttcatccagctcacctcctcgtgccccggctctgctgtgccgcccactgtgccattggtgacattctctggctcggtacacaggtaggagtaaaagccctctgacttgagcatgatgagcagcgagccccagcccaggaggactgccgagaagaggaggttctccagcacggccgtgcaggccatccaccagcggcgccgatgggcagtggccagggtgggcgccatggtgcggcgcggcgcggctccggctccggctccggctctgcaccaccgctgccctccgctacgacagagccgccccggccaggcagggagacgtctcccgcagctcactccgaggtaaactgaggcatggaggcaagaaggggctaacgcatgctcagggccgtggaactagtcctggcctgcagcaggactgacatcgcctggggccagcatggaacgcagcgtgaggtgggcaggggcagatccgagggctgcctctcccagggaccctgacaggtgccctcccgcccgcgcccgagacccttccccagagctggtttcttcaaccacaagatcagcgcccagacct

SEQ ID NO: 10866 - RNA, 7697 nt, Homo sapiens
  source 1..7697: mol_type = other RNA
ctgaatagctgggactacaggtacccaccaccacgcccagctaatttttttttttcgtatttttagtagagatggggtttcactgtgttagccacgttggtctcgatctcctgaccttgtgatccgcccgcctcagcctcccaaagtgctgggattacaggcgtgagccactgcgcccggccctaatttttgtatttttagtagagttgaggtttcaccatgttggtcaggctggtctcaaacccctgacctcaagtgatccaccccgcccccgcttcggcctcccaaagcactgggattacagggatgagccacctcgctgggaccagaccttactttcttgacttggccacaagtctgtcctgctcagagctgctgaaagtggctctcctgttgtatgggcttgggtgtggtgtggtggccctttccctgtcccagctgccttcttcctgggcactgaaaacgatgctaccattgtttttttttttttttttgagacggagtctcgctctgtcgcccaggctggagtgcagtggcgggatctcggctcactgcaagctccgcctcccgggttcacaccattctcctgcctcagcctcccaagtagctgggactacaggcgcccgccactacgcccggctaattttttgtatttttagtagagacggggtttcaccgttttagccgggatggtcttgatctcctgacctcgtgatccgcccgcctcggcctcccaaagtgctgggattacaggcgtgagccaccgcgcccggccaaatgctaccattgttaagtgccaggcgtcccaccatgcgggtcttcactgcgtatccacgtagctgcaccacgcaggcattctttcctcccttttgcagatgatggcaccaaagttcaagactcgcccagggccaccaagacagtcctctagactttggtcttccctccttgcctcctcggcctggggtggtggcgcctcggtctgagaagggtcgaggtctgggtgctgctagtggccctggctcagtctcagagctgcccggagggggtgaggatggctaacttaaggagcacaggcagaggcttcctgctggcaggaagagggctgagctgcggaaggccacccaggtggagtgtgctgcacctccttcagtggccttcaggagctctgtcctcacccagggattggggtgagtcagggcatggggaaacaggctcacagagcccacctgctcaccctgaccaccccaccccaggggaccccaggctcctaactctcagaatcccacagtctgtattggcggaagacgggctggcacccttgagttaggcccccagtcgttggcacagataaggggagctgctgctgaaggagcccgacggctgattctgtggaggcttctcagagctcctggcaggagcccctcaccgcaggaggcccacaacccctcccagctgcatatcggctcacattcacgcggctgccacacaagtgcgtcggaaactccacttggctgaacgtgattgtgctgctgtctgggacagtcttatgcacgtgagcccaatactggatgtcccgccattttcagccctggggcctatggcaaagtgacgcccccctcggagtgcacggcaggcaaggaaggtttaaacggaagttctgaccaggacgatgctgggtgcaagaggggacggggatggagcaaaacagaaaggatccaccagggcctgcaaccacgtctttggccccggtgaggggtgggaccttgtgtataggtccaggcagcagcagctgcagacagaggcctagagggtttggagaaggccgaccacaaagacacgcctagaccccagagtctagtgaggagagggactgggggcagtgtttcggcagcagacccagacccagactcagacccaagcccccctcctcactgatcaaaaccccaagggcagggagcccttcctgctccttcccgccagagcctggaggatgaggggcagacgggaggcccggccactggtgcctgctcctttgatcagctgtagtcccttccccttcacagggcacttgtcttgctggttggggtcaccagggattgctcccccaagtacccatcagcctccagggcccaaatgattccatgcagtagctctctccccctcttctgagaaggctcttggctcccagaaacggaaaccatgcctgggcctgctccccttccttgggctgtgacccccctgccacagaggccccccccccgccacagaggtcccccctgccacagaggtccccctgccacagaggcctggtggcccctgagctgctgctccgagtggaatgtcctggtctagaggcccttggctgctccagtgtcttaagacccatatatgagtgctggctctgaccttgaacaagctcctccatcgctccaggcctcgtttttcaggtgtatatgatgatagtatctctaggcctcgtttttcagttgtaaagcagggatgatcatatgtgtttaactcccagattgttatcaagtcaaggacaacaataggaaaacatgtcacctgtcagctccacacaaggcaaagtaggatgggtgacccctgactagggggtgggagtgcagggggcacccgacccatctggccagccacagcctctgtaccctgctcgcattttcaggcctcaatccccaagcactgttggccctggactgtttccccccctcaattctgtttctcaatgcctgcttcttcccagtaagtgccacaccctgagggtgggtgggagagtgaggcagcactgcccactttggctgggactgggcactgctggggacagcacgggccacgtcttccccatctcaagactggctttttggctaggcattgtgactcacgcctgtaatctcagcactttgggaggctgaggtgggagaattgcttcagcccaggagttccagaccagcctgggcaaaatagcaagaattcatctttatgaaaaagaaaaaaaaaattagccaggcatggtggcacacacttatagtcccagatacttaggaggccgaggtgggaggatcccttgagcccatgagttggaggccgtggtgagctatcagttgcaccactgcactccagcctggatggcagagcaagaccccaactcaaaaaaaaaaaaaaaaaaaaaaaggcggccttttcccagctggcagcaccctggctagttagggtttctccgaatctgcaactcctgtgtgatggcgggtctcaaatgctggcagcagagtcaccggtcagcggcaagacctggagtctccatttggaaccagcacccgggagcctctgctgggggtgatcatggagccgcacgtggaggctggtggctctgatggttcgagccgttcctcggcagcacagcacacccgctcctgaggagccacggagctcatgagcgttggcaaagtgctgtcagtgctggctgtaaggaaacaggcttgacttttaactcagcctttcccaaacttgactataatactttcttgaaaatcagaataaccactaacatcacaaaacgagtgttctcaggagtgggcatgtttatctcgttctctttttttttttctttttgagacggagcctcgctctgttgcccaggctggagtgcaatggtgcgatctcgactcacggcaatctccgtctccccggttcaagcgattctcctgcctcaggctcccgagtagttgggattacaggcgcacgccaccacgcccgattaatgtttatttttagtacagacggggtttctccatgttggtcaggatggtctcgaactcctgacctcaggtgagcctcctgccttggcctcccaaagtgctgggattataggcgtgagccaccacgcccagtctttttttaaatatttgagtgaaataaagcctaggagatatgtgttccaggcgcccaagctgttaatgtggagcttgaatgtggcctggacctgccctttcctcttctcctttcatccccctccctgccgcccacatcctgaactgctctgagcctgcagaagaacccagcgggaatcttcagggttgtggaagggtgtagggatggaaagggaccaggattcgcctgtttggctgggaaaatcggtagaggagggtggctcacacttctaagatgtctgcacaagcccagtttgtttgggggttggggaggaaggtcttttcctggcccactgtccctcccgagtcagcagtcccccagagagacgaagagcagctgggcacggctggagctggtcggtggcagagaatcttgtcctgccttttcttctcaagctcaaaataggcacatgcagctattaactgatatgccagaaggggcatcccttacccggaggaaaatggatttattgctttataaaaaagaagtctaataaaactgaagagaaaataactaaaaatccaaacacaactcacccctctaagcacgcccaggaggtctcaagacacacttctgggggcagtcaaggtgggcgggttggtgggccaggcggacgggcctcccccgtcatcagctccagggccccacggagcccgccggcagggggtgctgtgggcctgtggccttggacaagctcctggccccacgccaggatggctcctgggcactggcccagctgcaggcctggcggctcccgcctggtcagtggggataagggctaactcctagagcccaccccgaccccacacacacctcggacccacccacgtccccaccccggcctggacctccacgtctgccggccacagcctttcgtccacctccacaaaagcagctgtgtgtatgtacggggtgccctggcggcggtcctcaaattcccttcaggtggcagacagaacgagggtgacagtgaaaacgtgtccgcggcattggccctcggggaggaggcgaggggtccacccagcccgctaaaccctctccagggcataagccaggtggggcttctccaccggcctccaacgggtgggcaggccctggacaggcgacagggggctggaattacaaaggaattagcaccgacaacaggaagcgggtccttccttcctcaggcagcctcaggctggccggggagggggtgggggccaggcgcgggcgagacagtgcaagcctttgtcctcaggcaggtacggctgtgggcatgcagccgaggggcaggtggcaggcaggggatggcagccccctctgctttggcaagaggcagaatccagacactggcgggagagcgcctgcctgccgggcgttcctggctcctgctgcaggcaccacagagaccccaggccccgggtccccggggggcggcagagcaaagtcagggcagcccctgcgttcggcaggagaaaacgcgcgtgtccggggccctctcccgtccttccaccacagagctccgaggcagggccccgggagggagcgtgaacgctggcacggagacggcgaaggtcctgggggtgcgtggggtactctggaggggcaggacaggggtcagtcactgaagcacaggcaggagaccgcagttccgaggcggcagccactacacgaaggcctcctggttggacgagccgttgattttgaggaagagtttgtcatcctcctgcctctgctgcagctgccgctccagctggcgccggtagcagatcaggtagagcgggaggcagaagcccagcaggctgagaaggagcagccccacgttcacccacagagggtctccctggagaggacccatcatggccagaaacagcggctgctgcagaagggcgaagagcgcgctgatcagagactgcagtcccgtgaggctgccgaactgggtggaggggtacacggcagcgtacaggcccccgacagcggagtggatgaatcctcgcacgattgtgtgcaggatgaaggagaggatctggagaggcaggttgggaatgaggcaggtcaccccaaagcccacgagcagcaggttggtgaaggcgaaggcccgcatggcattagtgatcttctggatctgccggtcccgcttcttctttttcttctcgccttggttggcgtctttctcctcgggctcctcggaggcgtcttcacactccttcagcctccagtccatgatgtagccaatgacgggggccgtcagcaggcacagcagctggagcacgccgaagatggaggtgtagaggccaaccgtggccatcactgtcttctggtcgccgctgaccaggaacttgaggatgttgttcatagcccccatgtagaagatgagccgcagctgcgtgacgcacatggtgaccaggctgagcagcaggatggggctgaacacgctgtgcatgaaggagggggccactgcggcatccggctggcacttcacctccaggtcgacggtggacaggcacagcttgtggccctcctgcagcgccacctgctccttggcactcctcatggagctgcccacactcaggcgccggcccaccgtggtcacctgcttgtagaactgcttccctgtgatcttgtggtcaaagcccagccagctgaacttgatcttcaccgagtagtccatgtcctccggccccgggaagggctcaaggggccagttaaagaagcagttgaggaaaaccagcccggagcagccggcccagaccacgaggacgacgatgaaggagacaccagcatcatagatgagcttgattcctggaaaggtgactgccgaggaggcgtaggacccaatcatcaaggcaataaacgtggaccgaaggtcgccgaacatgttgggcagtgttaatgaggtgaaggtcatacacatcccaccaaagccattcagagccagggcgatgaagatgagcacggagagagcgtttggtttacttgctccgtacgcaatcagcaagcaggaaaccgcgaagcaggcgctgcccagcagcctgagcttcctcgggccatacttgtccatgacgatacccaggggcagggtgatggcactgagcagaaaggagcccacagtgaaggccaaatttagcatctcgtcctgggcctggcagctgagccagccgttcatccagctcacctcctcgtgccccggctctgctgtgccgcccactgtgccattggtgacattctctggctcggtacacaggtaggagtaaaagccctctgacttgagcatgatgagcagcgagccccagcccaggaggactgccgagaagaggaggttctccagcacggccgtgcaggccatccaccagcggcgccgatgggcagtggccagggtgggcgccatggtgcggcgcggcgcggctccggctccggctccggctctgcaccacctgggacaccccgagcccgcggccggctcgtaccgctgccctccgctacgacagagccgccccggccaggcagggagacgtctcccgcagctcactccgaggtaaactgaggcatggaggcaagaaggggctaacgcatgctcagggccgtggaactagtcctggcctgcagcaggactgacatcgcctggggccagcatggaacgcagcgtgaggtgggcaggggcagatccgagggctgcctctcccagggaccctgacaggtgccctcccgcccgcgcccgagacccttccccagagctggtttcttcaaccacaagatcagcgcccagacct

SEQ ID NO: 10867 - RNA, 7097 nt, Homo sapiens
  source 1..7097: mol_type = other RNA
ctgaatagctgggactacaggtacccaccaccacgcccagctaatttttttttttcgtatttttagtagagatggggtttcactgtgttagccacgttggtctcgatctcctgaccttgtgatccgcccgcctcagcctcccaaagtgctgggattacaggcgtgagccactgcgcccggccctaatttttgtatttttagtagagttgaggtttcaccatgttggtcaggctggtctcaaacccctgacctcaagtgatccaccccgcccccgcttcggcctcccaaagcactgggattacagggatgagccacctcgctgggaccagaccttactttcttgacttggccacaagtctgtcctgctcagagctgctgaaagtggctctcctgttgtatgggcttgggtgtggtgtggtggccctttccctgtcccagctgccttcttcctgggcactgaaaacgatgctaccattgtttttttttttttttttgagacggagtctcgctctgtcgcccaggctggagtgcagtggcgggatctcggctcactgcaagctccgcctcccgggttcacaccattctcctgcctcagcctcccaagtagctgggactacaggcgcccgccactacgcccggctaattttttgtatttttagtagagacggggtttcaccgttttagccgggatggtcttgatctcctgacctcgtgatccgcccgcctcggcctcccaaagtgctgggattacaggcgtgagccaccgcgcccggccaaatgctaccattgttaagtgccaggcgtcccaccatgcgggtcttcactgcgtatccacgtagctgcaccacgcaggcattctttcctcccttttgcagatgatggcaccaaagttcaagactcgcccagggccaccaagacagtcctctagactttggtcttccctccttgcctcctcggcctggggtggtggcgcctcggtctgagaagggtcgaggtctgggtgctgctagtggccctggctcagtctcagagctgcccggagggggtgaggatggctaacttaaggagcacaggcagaggcttcctgctggcaggaagagggctgagctgcggaaggccacccaggtggagtgtgctgcacctccttcagtggccttcaggagctctgtcctcacccagggattggggtgagtcagggcatggggaaacaggctcacagagcccacctgctcaccctgaccaccccaccccaggggaccccaggctcctaactctcagaatcccacagtctgtattggcggaagacgggctggcacccttgagttaggcccccagtcgttggcacagataaggggagctgctgctgaaggagcccgacggctgattctgtggaggcttctcagagctcctggcaggagcccctcaccgcaggaggcccacaacccctcccagctgcatatcggctcacattcacgcggctgccacacaagtgcgtcggaaactccacttggctgaacgtgattgtgctgctgtctgggacagtcttatgcacgtgagcccaatactggatgtcccgccattttcagccctggggcctatggcaaagtgacgcccccctcggagtgcacggcaggcaaggaaggtttaaacggaagttctgaccaggacgatgctgggtgcaagaggggacggggatggagcaaaacagaaaggatccaccagggcctgcaaccacgtctttggccccggtgaggggtgggaccttgtgtataggtccaggcagcagcagctgcagacagaggcctagagggtttggagaaggccgaccacaaagacacgcctagaccccagagtctagtgaggagagggactgggggcagtgtttcggcagcagacccagacccagactcagacccaagcccccctcctcactgatcaaaaccccaagggcagggagcccttcctgctccttcccgccagagcctggaggatgaggggcagacgggaggcccggccactggtgcctgctcctttgatcagctgtagtcccttccccttcacagggcacttgtcttgctggttggggtcaccagggattgctcccccaagtacccatcagcctccagggcccaaatgattccatgcagtagctctctccccctcttctgagaaggctcttggctcccagaaacggaaaccatgcctgggcctgctccccttccttgggctgtgacccccctgccacagaggccccccccccgccacagaggtcccccctgccacagaggtccccctgccacagaggcctggtggcccctgagctgctgctccgagtggaatgtcctggtctagaggcccttggctgctccagtgtcttaagacccatatatgagtgctggctctgaccttgaacaagctcctccatcgctccaggcctcgtttttcaggtgtatatgatgatagtatctctaggcctcgtttttcagttgtaaagcagggatgatcatatgtgtttaactcccagattgttatcaagtcaaggacaacaataggaaaacatgtcacctgtcagctccacacaaggcaaagtaggatgggtgacccctgactagggggtgggagtgcagggggcacccgacccatctggccagccacagcctctgtaccctgctcgcattttcaggcctcaatccccaagcactgttggccctggactgtttccccccctcaattctgtttctcaatgcctgcttcttcccagtaagtgccacaccctgagggtgggtgggagagtgaggcagcactgcccactttggctgggactgggcactgctggggacagcacgggccacgtcttccccatctcaagactggctttttggctaggcattgtgactcacgcctgtaatctcagcactttgggaggctgaggtgggagaattgcttcagcccaggagttccagaccagcctgggcaaaatagcaagaattcatctttatgaaaaagaaaaaaaaaattagccaggcatggtggcacacacttatagtcccagatacttaggaggccgaggtgggaggatcccttgagcccatgagttggaggccgtggtgagctatcagttgcaccactgcactccagcctggatggcagagcaagaccccaactcaaaaaaaaaaaaaaaaaaaaaaaggcggccttttcccagctggcagcaccctggctagttagggtttctccgaatctgcaactcctgtgtgatggcgggtctcaaatgctggcagcagagtcaccggtcagcggcaagacctggagtctccatttggaaccagcacccgggagcctctgctgggggtgatcatggagccgcacgtggaggctggtggctctgatggttcgagccgttcctcggcagcacagcacacccgctcctgaggagccacggagctcatgagcgttggcaaagtgctgtcagtgctggctgtaaggaaacaggcttgacttttaactcagcctttcccaaacttgactataatactttcttgaaaatcagaataaccactaacatcacaaaacgagtgttctcaggagtgggcatgtttatctcgttctctttttttttttctttttgagacggagcctcgctctgttgcccaggctggagtgcaatggtgcgatctcgactcacggcaatctccgtctccccggttcaagcgattctcctgcctcaggctcccgagtagttgggattacaggcgcacgccaccacgcccgattaatgtttatttttagtacagacggggtttctccatgttggtcaggatggtctcgaactcctgacctcaggtgagcctcctgccttggcctcccaaagtgctgggattataggcgtgagccaccacgcccagtctttttttaaatatttgagtgaaataaagcctaggagatatgtgttccaggcgcccaagctgttaatgtggagcttgaatgtggcctggacctgccctttcctcttctcctttcatccccctccctgccgcccacatcctgaactgctctgagcctgcagaagaacccagcgggaatcttcagggttgtggaagggtgtagggatggaaagggaccaggattcgcctgtttggctgggaaaatcggtagaggagggtggctcacacttctaagatgtctgcacaagcccagtttgtttgggggttggggaggaaggtcttttcctggcccactgtccctcccgagtcagcagtcccccagagagacgaagagcagctgggcacggctggagctggtcggtggcagagaatcttgtcctgccttttcttctcaagctcaaaataggcacatgcagctattaactgatatgccagaaggggcatcccttacccggaggaaaatggatttattgctttataaaaaagaagtctaataaaactgaagagaaaataactaaaaatccaaacacaactcacccctctaagcacgcccaggaggtctcaagacacacttctgggggcagtcaaggtgggcgggttggtgggccaggcggacgggcctcccccgtcatcagctccagggccccacggagcccgccggcagggggtgctgtgggcctgtggccttggacaagctcctggccccacgccaggatggctcctgggcactggcccagctgcaggcctggcggctcccgcctggtcagtggggataagggctaactcctagagcccaccccgaccccacacacacctcggacccacccacgtccccaccccggcctggacctccacgtctgccggccacagcctttcgtccacctccacaaaagcagctgtgtgtatgtacggggtgccctggcggcggtcctcaaattcccttcaggtggcagacagaacgagggtgacagtgaaaacgtgtccgcggcattggccctcggggaggaggcgaggggtccacccagcccgctaaaccctctccagggcataagccaggtggggcttctccaccggcctccaacgggtgggcaggccctggacaggcgacagggggctggaattacaaaggaattagcaccgacaacaggaagcgggtccttccttcctcaggcagcctcaggctggccggggagggggtgggggccaggcgcgggcgagacagtgcaagcctttgtcctcaggcaggtacggctgtgggcatgcagccgaggggcaggtggcaggcaggggatggcagccccctctgctttggcaagaggcagaatccagacactggcgggagagcgcctgcctgccgggcgttcctggctcctgctgcaggcaccacagagaccccaggccccgggtccccggggggcggcagagcaaagtcagggcagcccctgcgttcggcaggagaaaacgcgcgtgtccggggccctctcccgtccttccaccacagagctccgaggcagggccccgggagggagcgtgaacgctggcacggagacggcgaaggtcctgggggtgcgtggggtactctggaggggcaggacaggggtcagtcactgaagcacaggcaggagaccgcagttccgaggcggcagccactacacgaaggcctcctggttggacgagccgttgattttgaggaagagtttgtcatcctcctgcctctgctgcagctgccgctccagctggcgccggtagcagatcaggtagagcgggaggcagaagcccagcaggctgagaaggagcagccccacgttcacccacagagggtctccctggagaggacccatcatggccagaaacagcggctgctgcagaagggcgaagagcgcgctgatcagagactgcagtcccgtgaggctgccgaactgggtggaggggtacacggcagcgtacaggcccccgacagcggagtggatgaatcctcgcacgattgtgtgcaggatgaaggagaggatctggagaggcaggttgggaatgaggcaggtcaccccaaagcccacgagcagcaggttggtgaaggcgaaggcccgcatggcattagtgatcttctggatctgccggtcccgcttcttctttttcttctcgccttggttggcgtctttctcctcgggctcctcggaggcgtcttcacactccttcagcctccagtccatgatgtagccaatgacgggggccgtcagcaggcacagcagctggagcacgccgaagatggaggtgtagaggccaactgtcttctggtcgccgctgaccaggaacttgaggatgttgttcatagcccccatgtagaagatgagccgcagctgcgtgacgcacatggtgaccaggctgagcagcaggatggggctgaacacgctgtgcatgaaggagggggccactgcggcatccggctggcacttcacctccaggtcgacggtggacaggcacagcttgtggccctcctgcagcgccacctgctccttggcactcctcatggagctgcccacactcaggcgccggcccaccgtggtcacctgcttgtagaactgcttccctgtgatcttgtggtcaaagcccagccagctgaacttgatcttcaccgagtagtccatgtcctccggccccgggaagggctcaaggggccagttaaagaagcagttgaggaaaaccagcccggagcagccggcccagaccacgaggacgacgatgaaggagacaccagcatcatagatgagcttgattcctggaaaggtgactgccgaggaggcgtaggacccaatcatcaaggcaataaacgtggaccgaaggtcgccgaacatgttgggcagctcctgctgttgccttcggctgacctccccatggtccagcgccacagcatcggatgggcttgcatttgcctgtggactcccgtaggtcatcctgacatctgggtcactccccacattccccctctcgctcactccgtccccagcttccctgcctccaccggtctcagctgcgcataatggctgttcgaagccgcggtgccggagtgagggctgagcgctgagcagagcgccctagcgcgggcctcgagggctggcggaggggaaggaccccaggaggggaaggaccagctttgct

SEQ ID NO: 10868 - RNA, 7390 nt, Homo sapiens
  source 1..7390: mol_type = other RNA
ctgaatagctgggactacaggtacccaccaccacgcccagctaatttttttttttcgtatttttagtagagatggggtttcactgtgttagccacgttggtctcgatctcctgaccttgtgatccgcccgcctcagcctcccaaagtgctgggattacaggcgtgagccactgcgcccggccctaatttttgtatttttagtagagttgaggtttcaccatgttggtcaggctggtctcaaacccctgacctcaagtgatccaccccgcccccgcttcggcctcccaaagcactgggattacagggatgagccacctcgctgggaccagaccttactttcttgacttggccacaagtctgtcctgctcagagctgctgaaagtggctctcctgttgtatgggcttgggtgtggtgtggtggccctttccctgtcccagctgccttcttcctgggcactgaaaacgatgctaccattgtttttttttttttttttgagacggagtctcgctctgtcgcccaggctggagtgcagtggcgggatctcggctcactgcaagctccgcctcccgggttcacaccattctcctgcctcagcctcccaagtagctgggactacaggcgcccgccactacgcccggctaattttttgtatttttagtagagacggggtttcaccgttttagccgggatggtcttgatctcctgacctcgtgatccgcccgcctcggcctcccaaagtgctgggattacaggcgtgagccaccgcgcccggccaaatgctaccattgttaagtgccaggcgtcccaccatgcgggtcttcactgcgtatccacgtagctgcaccacgcaggcattctttcctcccttttgcagatgatggcaccaaagttcaagactcgcccagggccaccaagacagtcctctagactttggtcttccctccttgcctcctcggcctggggtggtggcgcctcggtctgagaagggtcgaggtctgggtgctgctagtggccctggctcagtctcagagctgcccggagggggtgaggatggctaacttaaggagcacaggcagaggcttcctgctggcaggaagagggctgagctgcggaaggccacccaggtggagtgtgctgcacctccttcagtggccttcaggagctctgtcctcacccagggattggggtgagtcagggcatggggaaacaggctcacagagcccacctgctcaccctgaccaccccaccccaggggaccccaggctcctaactctcagaatcccacagtctgtattggcggaagacgggctggcacccttgagttaggcccccagtcgttggcacagataaggggagctgctgctgaaggagcccgacggctgattctgtggaggcttctcagagctcctggcaggagcccctcaccgcaggaggcccacaacccctcccagctgcatatcggctcacattcacgcggctgccacacaagtgcgtcggaaactccacttggctgaacgtgattgtgctgctgtctgggacagtcttatgcacgtgagcccaatactggatgtcccgccattttcagccctggggcctatggcaaagtgacgcccccctcggagtgcacggcaggcaaggaaggtttaaacggaagttctgaccaggacgatgctgggtgcaagaggggacggggatggagcaaaacagaaaggatccaccagggcctgcaaccacgtctttggccccggtgaggggtgggaccttgtgtataggtccaggcagcagcagctgcagacagaggcctagagggtttggagaaggccgaccacaaagacacgcctagaccccagagtctagtgaggagagggactgggggcagtgtttcggcagcagacccagacccagactcagacccaagcccccctcctcactgatcaaaaccccaagggcagggagcccttcctgctccttcccgccagagcctggaggatgaggggcagacgggaggcccggccactggtgcctgctcctttgatcagctgtagtcccttccccttcacagggcacttgtcttgctggttggggtcaccagggattgctcccccaagtacccatcagcctccagggcccaaatgattccatgcagtagctctctccccctcttctgagaaggctcttggctcccagaaacggaaaccatgcctgggcctgctccccttccttgggctgtgacccccctgccacagaggccccccccccgccacagaggtcccccctgccacagaggtccccctgccacagaggcctggtggcccctgagctgctgctccgagtggaatgtcctggtctagaggcccttggctgctccagtgtcttaagacccatatatgagtgctggctctgaccttgaacaagctcctccatcgctccaggcctcgtttttcaggtgtatatgatgatagtatctctaggcctcgtttttcagttgtaaagcagggatgatcatatgtgtttaactcccagattgttatcaagtcaaggacaacaataggaaaacatgtcacctgtcagctccacacaaggcaaagtaggatgggtgacccctgactagggggtgggagtgcagggggcacccgacccatctggccagccacagcctctgtaccctgctcgcattttcaggcctcaatccccaagcactgttggccctggactgtttccccccctcaattctgtttctcaatgcctgcttcttcccagtaagtgccacaccctgagggtgggtgggagagtgaggcagcactgcccactttggctgggactgggcactgctggggacagcacgggccacgtcttccccatctcaagactggctttttggctaggcattgtgactcacgcctgtaatctcagcactttgggaggctgaggtgggagaattgcttcagcccaggagttccagaccagcctgggcaaaatagcaagaattcatctttatgaaaaagaaaaaaaaaattagccaggcatggtggcacacacttatagtcccagatacttaggaggccgaggtgggaggatcccttgagcccatgagttggaggccgtggtgagctatcagttgcaccactgcactccagcctggatggcagagcaagaccccaactcaaaaaaaaaaaaaaaaaaaaaaaggcggccttttcccagctggcagcaccctggctagttagggtttctccgaatctgcaactcctgtgtgatggcgggtctcaaatgctggcagcagagtcaccggtcagcggcaagacctggagtctccatttggaaccagcacccgggagcctctgctgggggtgatcatggagccgcacgtggaggctggtggctctgatggttcgagccgttcctcggcagcacagcacacccgctcctgaggagccacggagctcatgagcgttggcaaagtgctgtcagtgctggctgtaaggaaacaggcttgacttttaactcagcctttcccaaacttgactataatactttcttgaaaatcagaataaccactaacatcacaaaacgagtgttctcaggagtgggcatgtttatctcgttctctttttttttttctttttgagacggagcctcgctctgttgcccaggctggagtgcaatggtgcgatctcgactcacggcaatctccgtctccccggttcaagcgattctcctgcctcaggctcccgagtagttgggattacaggcgcacgccaccacgcccgattaatgtttatttttagtacagacggggtttctccatgttggtcaggatggtctcgaactcctgacctcaggtgagcctcctgccttggcctcccaaagtgctgggattataggcgtgagccaccacgcccagtctttttttaaatatttgagtgaaataaagcctaggagatatgtgttccaggcgcccaagctgttaatgtggagcttgaatgtggcctggacctgccctttcctcttctcctttcatccccctccctgccgcccacatcctgaactgctctgagcctgcagaagaacccagcgggaatcttcagggttgtggaagggtgtagggatggaaagggaccaggattcgcctgtttggctgggaaaatcggtagaggagggtggctcacacttctaagatgtctgcacaagcccagtttgtttgggggttggggaggaaggtcttttcctggcccactgtccctcccgagtcagcagtcccccagagagacgaagagcagctgggcacggctggagctggtcggtggcagagaatcttgtcctgccttttcttctcaagctcaaaataggcacatgcagctattaactgatatgccagaaggggcatcccttacccggaggaaaatggatttattgctttataaaaaagaagtctaataaaactgaagagaaaataactaaaaatccaaacacaactcacccctctaagcacgcccaggaggtctcaagacacacttctgggggcagtcaaggtgggcgggttggtgggccaggcggacgggcctcccccgtcatcagctccagggccccacggagcccgccggcagggggtgctgtgggcctgtggccttggacaagctcctggccccacgccaggatggctcctgggcactggcccagctgcaggcctggcggctcccgcctggtcagtggggataagggctaactcctagagcccaccccgaccccacacacacctcggacccacccacgtccccaccccggcctggacctccacgtctgccggccacagcctttcgtccacctccacaaaagcagctgtgtgtatgtacggggtgccctggcggcggtcctcaaattcccttcaggtggcagacagaacgagggtgacagtgaaaacgtgtccgcggcattggccctcggggaggaggcgaggggtccacccagcccgctaaaccctctccagggcataagccaggtggggcttctccaccggcctccaacgggtgggcaggccctggacaggcgacagggggctggaattacaaaggaattagcaccgacaacaggaagcgggtccttccttcctcaggcagcctcaggctggccggggagggggtgggggccaggcgcgggcgagacagtgcaagcctttgtcctcaggcaggtacggctgtgggcatgcagccgaggggcaggtggcaggcaggggatggcagccccctctgctttggcaagaggcagaatccagacactggcgggagagcgcctgcctgccgggcgttcctggctcctgctgcaggcaccacagagaccccaggccccgggtccccggggggcggcagagcaaagtcagggcagcccctgcgttcggcaggagaaaacgcgcgtgtccggggccctctcccgtccttccaccacagagctccgaggcagggccccgggagggagcgtgaacgctggcacggagacggcgaaggtcctgggggtgcgtggggtactctggaggggcaggacaggggtcagtcactgaagcacaggcaggagaccgcagttccgaggcggcagccactacacgaaggcctcctggttggacgagccgttgattttgaggaagagtttgtcatcctcctgcctctgctgcagctgccgctccagctggcgccggtagcagatcaggtagagcgggaggcagaagcccagcaggctgagaaggagcagccccacgttcacccacagagggtctccctggagaggacccatcatggccagaaacagcggctgctgcagaagggcgaagagcgcgctgatcagagactgcagtcccgtgaggctgccgaactgggtggaggggtacacggcagcgtacaggcccccgacagcggagtggatgaatcctcgcacgattgtgtgcaggatgaaggagaggatctggagaggcaggttgggaatgaggcaggtcaccccaaagcccacgagcagcaggttggtgaaggcgaaggcccgcatggcattagtgatcttctggatctgccggtcccgcttcttctttttcttctcgccttggttggcgtctttctcctcgggctcctcggaggcgtcttcacactccttcagcctccagtccatgatgtagccaatgacgggggccgtcagcaggcacagcagctggagcacgccgaagatggaggtgtagaggccaactgtcttctggtcgccgctgaccaggaacttgaggatgttgttcatagcccccatgtagaagatgagccgcagctgcgtgacgcacatggtgaccaggctgagcagcaggatggggctgaacacgctgtgcatgaaggagggggccactgcggcatccggctggcacttcacctccaggtcgacggtggacaggcacagcttgtggccctcctgcagcgccacctgctccttggcactcctcatggagctgcccacactcaggcgccggcccaccgtggtcacctgcttgtagaactgcttccctgtgatcttgtggtcaaagcccagccagctgaacttgatcttcaccgagtagtccatgtcctccggccccgggaagggctcaaggggccagttaaagaagcagttgaggaaaaccagcccggagcagccggcccagaccacgaggacgacgatgaaggagacaccagcatcatagatgagcttgattcctggaaaggtgactgccgaggaggcgtaggacccaatcatcaaggcaataaacgtggaccgaaggtcgccgaacatgttgggcagtgttaatgaggtgaaggtcatacacatcccaccaaagccattcagagccagggcgatgaagatgagcacggagagagcgtttggtttacttgctccgtacgcaatcagcaagcaggaaaccgcgaagcaggcgctgcccagcagcctgagcttcctcgggccatacttgtccatgacgatacccaggggcagggtgatggcactgagcagaaaggagcccacagtgaaggccaaatttagcatctcgtcctgggcctggcagctgagccagccgttcatccagctcacctcctcgtgccccggctctgctgtgccgcccactgtgccattggtgacattctctggctcggtacacaggtaggagtaaaagccctctgacttgagcatgatgagcagcgagccccagcccaggaggactgccgagaagaggaggttctccagcacggccgtgcaggccatccaccagcggcgccgatgggcagtggccagggtgggcgccatggtgcggcgcggcgcggctccggctccggctccggctctgcaccacccggctcctccggcgtgtgtcgggcccgcccggcgcctttt

SEQ ID NO: 10869 - RNA, 7620 nt, Homo sapiens
  source 1..7620: mol_type = other RNA
ctgaatagctgggactacaggtacccaccaccacgcccagctaatttttttttttcgtatttttagtagagatggggtttcactgtgttagccacgttggtctcgatctcctgaccttgtgatccgcccgcctcagcctcccaaagtgctgggattacaggcgtgagccactgcgcccggccctaatttttgtatttttagtagagttgaggtttcaccatgttggtcaggctggtctcaaacccctgacctcaagtgatccaccccgcccccgcttcggcctcccaaagcactgggattacagggatgagccacctcgctgggaccagaccttactttcttgacttggccacaagtctgtcctgctcagagctgctgaaagtggctctcctgttgtatgggcttgggtgtggtgtggtggccctttccctgtcccagctgccttcttcctgggcactgaaaacgatgctaccattgtttttttttttttttttgagacggagtctcgctctgtcgcccaggctggagtgcagtggcgggatctcggctcactgcaagctccgcctcccgggttcacaccattctcctgcctcagcctcccaagtagctgggactacaggcgcccgccactacgcccggctaattttttgtatttttagtagagacggggtttcaccgttttagccgggatggtcttgatctcctgacctcgtgatccgcccgcctcggcctcccaaagtgctgggattacaggcgtgagccaccgcgcccggccaaatgctaccattgttaagtgccaggcgtcccaccatgcgggtcttcactgcgtatccacgtagctgcaccacgcaggcattctttcctcccttttgcagatgatggcaccaaagttcaagactcgcccagggccaccaagacagtcctctagactttggtcttccctccttgcctcctcggcctggggtggtggcgcctcggtctgagaagggtcgaggtctgggtgctgctagtggccctggctcagtctcagagctgcccggagggggtgaggatggctaacttaaggagcacaggcagaggcttcctgctggcaggaagagggctgagctgcggaaggccacccaggtggagtgtgctgcacctccttcagtggccttcaggagctctgtcctcacccagggattggggtgagtcagggcatggggaaacaggctcacagagcccacctgctcaccctgaccaccccaccccaggggaccccaggctcctaactctcagaatcccacagtctgtattggcggaagacgggctggcacccttgagttaggcccccagtcgttggcacagataaggggagctgctgctgaaggagcccgacggctgattctgtggaggcttctcagagctcctggcaggagcccctcaccgcaggaggcccacaacccctcccagctgcatatcggctcacattcacgcggctgccacacaagtgcgtcggaaactccacttggctgaacgtgattgtgctgctgtctgggacagtcttatgcacgtgagcccaatactggatgtcccgccattttcagccctggggcctatggcaaagtgacgcccccctcggagtgcacggcaggcaaggaaggtttaaacggaagttctgaccaggacgatgctgggtgcaagaggggacggggatggagcaaaacagaaaggatccaccagggcctgcaaccacgtctttggccccggtgaggggtgggaccttgtgtataggtccaggcagcagcagctgcagacagaggcctagagggtttggagaaggccgaccacaaagacacgcctagaccccagagtctagtgaggagagggactgggggcagtgtttcggcagcagacccagacccagactcagacccaagcccccctcctcactgatcaaaaccccaagggcagggagcccttcctgctccttcccgccagagcctggaggatgaggggcagacgggaggcccggccactggtgcctgctcctttgatcagctgtagtcccttccccttcacagggcacttgtcttgctggttggggtcaccagggattgctcccccaagtacccatcagcctccagggcccaaatgattccatgcagtagctctctccccctcttctgagaaggctcttggctcccagaaacggaaaccatgcctgggcctgctccccttccttgggctgtgacccccctgccacagaggccccccccccgccacagaggtcccccctgccacagaggtccccctgccacagaggcctggtggcccctgagctgctgctccgagtggaatgtcctggtctagaggcccttggctgctccagtgtcttaagacccatatatgagtgctggctctgaccttgaacaagctcctccatcgctccaggcctcgtttttcaggtgtatatgatgatagtatctctaggcctcgtttttcagttgtaaagcagggatgatcatatgtgtttaactcccagattgttatcaagtcaaggacaacaataggaaaacatgtcacctgtcagctccacacaaggcaaagtaggatgggtgacccctgactagggggtgggagtgcagggggcacccgacccatctggccagccacagcctctgtaccctgctcgcattttcaggcctcaatccccaagcactgttggccctggactgtttccccccctcaattctgtttctcaatgcctgcttcttcccagtaagtgccacaccctgagggtgggtgggagagtgaggcagcactgcccactttggctgggactgggcactgctggggacagcacgggccacgtcttccccatctcaagactggctttttggctaggcattgtgactcacgcctgtaatctcagcactttgggaggctgaggtgggagaattgcttcagcccaggagttccagaccagcctgggcaaaatagcaagaattcatctttatgaaaaagaaaaaaaaaattagccaggcatggtggcacacacttatagtcccagatacttaggaggccgaggtgggaggatcccttgagcccatgagttggaggccgtggtgagctatcagttgcaccactgcactccagcctggatggcagagcaagaccccaactcaaaaaaaaaaaaaaaaaaaaaaaggcggccttttcccagctggcagcaccctggctagttagggtttctccgaatctgcaactcctgtgtgatggcgggtctcaaatgctggcagcagagtcaccggtcagcggcaagacctggagtctccatttggaaccagcacccgggagcctctgctgggggtgatcatggagccgcacgtggaggctggtggctctgatggttcgagccgttcctcggcagcacagcacacccgctcctgaggagccacggagctcatgagcgttggcaaagtgctgtcagtgctggctgtaaggaaacaggcttgacttttaactcagcctttcccaaacttgactataatactttcttgaaaatcagaataaccactaacatcacaaaacgagtgttctcaggagtgggcatgtttatctcgttctctttttttttttctttttgagacggagcctcgctctgttgcccaggctggagtgcaatggtgcgatctcgactcacggcaatctccgtctccccggttcaagcgattctcctgcctcaggctcccgagtagttgggattacaggcgcacgccaccacgcccgattaatgtttatttttagtacagacggggtttctccatgttggtcaggatggtctcgaactcctgacctcaggtgagcctcctgccttggcctcccaaagtgctgggattataggcgtgagccaccacgcccagtctttttttaaatatttgagtgaaataaagcctaggagatatgtgttccaggcgcccaagctgttaatgtggagcttgaatgtggcctggacctgccctttcctcttctcctttcatccccctccctgccgcccacatcctgaactgctctgagcctgcagaagaacccagcgggaatcttcagggttgtggaagggtgtagggatggaaagggaccaggattcgcctgtttggctgggaaaatcggtagaggagggtggctcacacttctaagatgtctgcacaagcccagtttgtttgggggttggggaggaaggtcttttcctggcccactgtccctcccgagtcagcagtcccccagagagacgaagagcagctgggcacggctggagctggtcggtggcagagaatcttgtcctgccttttcttctcaagctcaaaataggcacatgcagctattaactgatatgccagaaggggcatcccttacccggaggaaaatggatttattgctttataaaaaagaagtctaataaaactgaagagaaaataactaaaaatccaaacacaactcacccctctaagcacgcccaggaggtctcaagacacacttctgggggcagtcaaggtgggcgggttggtgggccaggcggacgggcctcccccgtcatcagctccagggccccacggagcccgccggcagggggtgctgtgggcctgtggccttggacaagctcctggccccacgccaggatggctcctgggcactggcccagctgcaggcctggcggctcccgcctggtcagtggggataagggctaactcctagagcccaccccgaccccacacacacctcggacccacccacgtccccaccccggcctggacctccacgtctgccggccacagcctttcgtccacctccacaaaagcagctgtgtgtatgtacggggtgccctggcggcggtcctcaaattcccttcaggtggcagacagaacgagggtgacagtgaaaacgtgtccgcggcattggccctcggggaggaggcgaggggtccacccagcccgctaaaccctctccagggcataagccaggtggggcttctccaccggcctccaacgggtgggcaggccctggacaggcgacagggggctggaattacaaaggaattagcaccgacaacaggaagcgggtccttccttcctcaggcagcctcaggctggccggggagggggtgggggccaggcgcgggcgagacagtgcaagcctttgtcctcaggcaggtacggctgtgggcatgcagccgaggggcaggtggcaggcaggggatggcagccccctctgctttggcaagaggcagaatccagacactggcgggagagcgcctgcctgccgggcgttcctggctcctgctgcaggcaccacagagaccccaggccccgggtccccggggggcggcagagcaaagtcagggcagcccctgcgttcggcaggagaaaacgcgcgtgtccggggccctctcccgtccttccaccacagagctccgaggcagggccccgggagggagcgtgaacgctggcacggagacggcgaaggtcctgggggtgcgtggggtactctggaggggcaggacaggggtcagtcactgaagcacaggcaggagaccgcagttccgaggcggcagccactacacgaaggcctcctggttggacgagccgttgattttgaggaagagtttgtcatcctcctgcctctgctgcagctgccgctccagctggcgccggtagcagatcaggtagagcgggaggcagaagcccagcaggctgagaaggagcagccccacgttcacccacagagggtctccctggagaggacccatcatggccagaaacagcggctgctgcagaagggcgaagagcgcgctgatcagagactgcagtcccgtgaggctgccgaactgggtggaggggtacacggcagcgtacaggcccccgacagcggagtggatgaatcctcgcacgattgtgtgcaggatgaaggagaggatctggagaggcaggttgggaatgaggcaggtcaccccaaagcccacgagcagcaggttggtgaaggcgaaggcccgcatggcattagtgatcttctggatctgccggtcccgcttcttctttttcttctcgccttggttggcgtctttctcctcgggctcctcggaggcgtcttcacactccttcagcctccagtccatgatgtagccaatgacgggggccgtcagcaggcacagcagctggagcacgccgaagatggaggtgtagaggccaactgtcttctggtcgccgctgaccaggaacttgaggatgttgttcatagcccccatgtagaagatgagccgcagctgcgtgacgcacatggtgaccaggctgagcagcaggatggggctgaacacgctgtgcatgaaggagggggccactgcggcatccggctggcacttcacctccaggtcgacggtggacaggcacagcttgtggccctcctgcagcgccacctgctccttggcactcctcatggagctgcccacactcaggcgccggcccaccgtggtcacctgcttgtagaactgcttccctgtgatcttgtggtcaaagcccagccagctgaacttgatcttcaccgagtagtccatgtcctccggccccgggaagggctcaaggggccagttaaagaagcagttgaggaaaaccagcccggagcagccggcccagaccacgaggacgacgatgaaggagacaccagcatcatagatgagcttgattcctggaaaggtgactgccgaggaggcgtaggacccaatcatcaaggcaataaacgtggaccgaaggtcgccgaacatgttgggcagtgttaatgaggtgaaggtcatacacatcccaccaaagccattcagagccagggcgatgaagatgagcacggagagagcgtttggtttacttgctccgtacgcaatcagcaagcaggaaaccgcgaagcaggcgctgcccagcagcctgagcttcctcgggccatacttgtccatgacgatacccaggggcagggtgatggcactgagcagaaaggagcccacagtgaaggccaaatttagcatctcgtcctgggcctggcagctgagccagccgttcatccagctcacctcctcgtgccccggctctgctgtgccgcccactgtgccattggtgacattctctggctcggtacacaggtaggagtaaaagccctctgacttgagcatgatgagcagcgagccccagcccaggaggactgccgagaagaggaggttctccagcacggccgtgcaggccatccaccagcggcgccgatgggcagtggccagggtgggcgccatggtgcggcgcggcgcggctccggctccggctccggctctgcaccaccgctgccctccgctacgacagagccgccccggccaggcagggagacgtctcccgcagctcactccgaggtaaactgaggcatggaggcaagaaggggctaacgcatgctcagggccgtggaactagtcctggcctgcagcaggactgacatcgcctggggccagcatggaacgcagcgtgaggtgggcaggggcagatccgagggctgcctctcccagggaccctgacaggtgccctcccgcccgcgcccgagacccttccccagagctgg

SEQ ID NO: 10870 - RNA, 7653 nt, Homo sapiens
  source 1..7653: mol_type = other RNA
ctgaatagctgggactacaggtacccaccaccacgcccagctaatttttttttttcgtatttttagtagagatggggtttcactgtgttagccacgttggtctcgatctcctgaccttgtgatccgcccgcctcagcctcccaaagtgctgggattacaggcgtgagccactgcgcccggccctaatttttgtatttttagtagagttgaggtttcaccatgttggtcaggctggtctcaaacccctgacctcaagtgatccaccccgcccccgcttcggcctcccaaagcactgggattacagggatgagccacctcgctgggaccagaccttactttcttgacttggccacaagtctgtcctgctcagagctgctgaaagtggctctcctgttgtatgggcttgggtgtggtgtggtggccctttccctgtcccagctgccttcttcctgggcactgaaaacgatgctaccattgtttttttttttttttttgagacggagtctcgctctgtcgcccaggctggagtgcagtggcgggatctcggctcactgcaagctccgcctcccgggttcacaccattctcctgcctcagcctcccaagtagctgggactacaggcgcccgccactacgcccggctaattttttgtatttttagtagagacggggtttcaccgttttagccgggatggtcttgatctcctgacctcgtgatccgcccgcctcggcctcccaaagtgctgggattacaggcgtgagccaccgcgcccggccaaatgctaccattgttaagtgccaggcgtcccaccatgcgggtcttcactgcgtatccacgtagctgcaccacgcaggcattctttcctcccttttgcagatgatggcaccaaagttcaagactcgcccagggccaccaagacagtcctctagactttggtcttccctccttgcctcctcggcctggggtggtggcgcctcggtctgagaagggtcgaggtctgggtgctgctagtggccctggctcagtctcagagctgcccggagggggtgaggatggctaacttaaggagcacaggcagaggcttcctgctggcaggaagagggctgagctgcggaaggccacccaggtggagtgtgctgcacctccttcagtggccttcaggagctctgtcctcacccagggattggggtgagtcagggcatggggaaacaggctcacagagcccacctgctcaccctgaccaccccaccccaggggaccccaggctcctaactctcagaatcccacagtctgtattggcggaagacgggctggcacccttgagttaggcccccagtcgttggcacagataaggggagctgctgctgaaggagcccgacggctgattctgtggaggcttctcagagctcctggcaggagcccctcaccgcaggaggcccacaacccctcccagctgcatatcggctcacattcacgcggctgccacacaagtgcgtcggaaactccacttggctgaacgtgattgtgctgctgtctgggacagtcttatgcacgtgagcccaatactggatgtcccgccattttcagccctggggcctatggcaaagtgacgcccccctcggagtgcacggcaggcaaggaaggtttaaacggaagttctgaccaggacgatgctgggtgcaagaggggacggggatggagcaaaacagaaaggatccaccagggcctgcaaccacgtctttggccccggtgaggggtgggaccttgtgtataggtccaggcagcagcagctgcagacagaggcctagagggtttggagaaggccgaccacaaagacacgcctagaccccagagtctagtgaggagagggactgggggcagtgtttcggcagcagacccagacccagactcagacccaagcccccctcctcactgatcaaaaccccaagggcagggagcccttcctgctccttcccgccagagcctggaggatgaggggcagacgggaggcccggccactggtgcctgctcctttgatcagctgtagtcccttccccttcacagggcacttgtcttgctggttggggtcaccagggattgctcccccaagtacccatcagcctccagggcccaaatgattccatgcagtagctctctccccctcttctgagaaggctcttggctcccagaaacggaaaccatgcctgggcctgctccccttccttgggctgtgacccccctgccacagaggccccccccccgccacagaggtcccccctgccacagaggtccccctgccacagaggcctggtggcccctgagctgctgctccgagtggaatgtcctggtctagaggcccttggctgctccagtgtcttaagacccatatatgagtgctggctctgaccttgaacaagctcctccatcgctccaggcctcgtttttcaggtgtatatgatgatagtatctctaggcctcgtttttcagttgtaaagcagggatgatcatatgtgtttaactcccagattgttatcaagtcaaggacaacaataggaaaacatgtcacctgtcagctccacacaaggcaaagtaggatgggtgacccctgactagggggtgggagtgcagggggcacccgacccatctggccagccacagcctctgtaccctgctcgcattttcaggcctcaatccccaagcactgttggccctggactgtttccccccctcaattctgtttctcaatgcctgcttcttcccagtaagtgccacaccctgagggtgggtgggagagtgaggcagcactgcccactttggctgggactgggcactgctggggacagcacgggccacgtcttccccatctcaagactggctttttggctaggcattgtgactcacgcctgtaatctcagcactttgggaggctgaggtgggagaattgcttcagcccaggagttccagaccagcctgggcaaaatagcaagaattcatctttatgaaaaagaaaaaaaaaattagccaggcatggtggcacacacttatagtcccagatacttaggaggccgaggtgggaggatcccttgagcccatgagttggaggccgtggtgagctatcagttgcaccactgcactccagcctggatggcagagcaagaccccaactcaaaaaaaaaaaaaaaaaaaaaaaggcggccttttcccagctggcagcaccctggctagttagggtttctccgaatctgcaactcctgtgtgatggcgggtctcaaatgctggcagcagagtcaccggtcagcggcaagacctggagtctccatttggaaccagcacccgggagcctctgctgggggtgatcatggagccgcacgtggaggctggtggctctgatggttcgagccgttcctcggcagcacagcacacccgctcctgaggagccacggagctcatgagcgttggcaaagtgctgtcagtgctggctgtaaggaaacaggcttgacttttaactcagcctttcccaaacttgactataatactttcttgaaaatcagaataaccactaacatcacaaaacgagtgttctcaggagtgggcatgtttatctcgttctctttttttttttctttttgagacggagcctcgctctgttgcccaggctggagtgcaatggtgcgatctcgactcacggcaatctccgtctccccggttcaagcgattctcctgcctcaggctcccgagtagttgggattacaggcgcacgccaccacgcccgattaatgtttatttttagtacagacggggtttctccatgttggtcaggatggtctcgaactcctgacctcaggtgagcctcctgccttggcctcccaaagtgctgggattataggcgtgagccaccacgcccagtctttttttaaatatttgagtgaaataaagcctaggagatatgtgttccaggcgcccaagctgttaatgtggagcttgaatgtggcctggacctgccctttcctcttctcctttcatccccctccctgccgcccacatcctgaactgctctgagcctgcagaagaacccagcgggaatcttcagggttgtggaagggtgtagggatggaaagggaccaggattcgcctgtttggctgggaaaatcggtagaggagggtggctcacacttctaagatgtctgcacaagcccagtttgtttgggggttggggaggaaggtcttttcctggcccactgtccctcccgagtcagcagtcccccagagagacgaagagcagctgggcacggctggagctggtcggtggcagagaatcttgtcctgccttttcttctcaagctcaaaataggcacatgcagctattaactgatatgccagaaggggcatcccttacccggaggaaaatggatttattgctttataaaaaagaagtctaataaaactgaagagaaaataactaaaaatccaaacacaactcacccctctaagcacgcccaggaggtctcaagacacacttctgggggcagtcaaggtgggcgggttggtgggccaggcggacgggcctcccccgtcatcagctccagggccccacggagcccgccggcagggggtgctgtgggcctgtggccttggacaagctcctggccccacgccaggatggctcctgggcactggcccagctgcaggcctggcggctcccgcctggtcagtggggataagggctaactcctagagcccaccccgaccccacacacacctcggacccacccacgtccccaccccggcctggacctccacgtctgccggccacagcctttcgtccacctccacaaaagcagctgtgtgtatgtacggggtgccctggcggcggtcctcaaattcccttcaggtggcagacagaacgagggtgacagtgaaaacgtgtccgcggcattggccctcggggaggaggcgaggggtccacccagcccgctaaaccctctccagggcataagccaggtggggcttctccaccggcctccaacgggtgggcaggccctggacaggcgacagggggctggaattacaaaggaattagcaccgacaacaggaagcgggtccttccttcctcaggcagcctcaggctggccggggagggggtgggggccaggcgcgggcgagacagtgcaagcctttgtcctcaggcaggtacggctgtgggcatgcagccgaggggcaggtggcaggcaggggatggcagccccctctgctttggcaagaggcagaatccagacactggcgggagagcgcctgcctgccgggcgttcctggctcctgctgcaggcaccacagagaccccaggccccgggtccccggggggcggcagagcaaagtcagggcagcccctgcgttcggcaggagaaaacgcgcgtgtccggggccctctcccgtccttccaccacagagctccgaggcagggccccgggagggagcgtgaacgctggcacggagacggcgaaggtcctgggggtgcgtggggtactctggaggggcaggacaggggtcagtcactgaagcacaggcaggagaccgcagttccgaggcggcagccactacacgaaggcctcctggttggacgagccgttgattttgaggaagagtttgtcatcctcctgcctctgctgcagctgccgctccagctggcgccggtagcagatcaggtagagcgggaggcagaagcccagcaggctgagaaggagcagccccacgttcacccacagagggtctccctggagaggacccatcatggccagaaacagcggctgctgcagaagggcgaagagcgcgctgatcagagactgcagtcccgtgaggctgccgaactgggtggaggggtacacggcagcgtacaggcccccgacagcggagtggatgaatcctcgcacgattgtgtgcaggatgaaggagaggatctggagaggcaggttgggaatgaggcaggtcaccccaaagcccacgagcagcaggttggtgaaggcgaaggcccgcatggcattagtgatcttctggatctgccggtcccgcttcttctttttcttctcgccttggttggcgtctttctcctcgggctcctcggaggcgtcttcacactccttcagcctccagtccatgatgtagccaatgacgggggccgtcagcaggcacagcagctggagcacgccgaagatggaggtgtagaggccaactgtcttctggtcgccgctgaccaggaacttgaggatgttgttcatagcccccatgtagaagatgagccgcagctgcgtgacgcacatggtgaccaggctgagcagcaggatggggctgaacacgctgtgcatgaaggagggggccactgcggcatccggctggcacttcacctccaggtcgacggtggacaggcacagcttgtggccctcctgcagcgccacctgctccttggcactcctcatggagctgcccacactcaggcgccggcccaccgtggtcacctgcttgtagaactgcttccctgtgatcttgtggtcaaagcccagccagctgaacttgatcttcaccgagtagtccatgtcctccggccccgggaagggctcaaggggccagttaaagaagcagttgaggaaaaccagcccggagcagccggcccagaccacgaggacgacgatgaaggagacaccagcatcatagatgagcttgattcctggaaaggtgactgccgaggaggcgtaggacccaatcatcaaggcaataaacgtggaccgaaggtcgccgaacatgttgggcagtgttaatgaggtgaaggtcatacacatcccaccaaagccattcagagccagggcgatgaagatgagcacggagagagcgtttggtttacttgctccgtacgcaatcagcaagcaggaaaccgcgaagcaggcgctgcccagcagcctgagcttcctcgggccatacttgtccatgacgatacccaggggcagggtgatggcactgagcagaaaggagcccacagtgaaggccaaatttagcatctcgtcctgggcctggcagctgagccagccgttcatccagctcacctcctcgtgccccggctctgctgtgccgcccactgtgccattggtgacattctctggctcggtacacaggtaggagtaaaagccctctgacttgagcatgatgagcagcgagccccagcccaggaggactgccgagaagaggaggttctccagcacggccgtgcaggccatccaccagcggcgccgatgggcagtggccagggtgggcgccatggtgcggcgcggcgcggctccggctccggctccggctctgcaccacctgggacaccccgagcccgcggccggctcgtaccgctgccctccgctacgacagagccgccccggccaggcagggagacgtctcccgcagctcactccgaggtaaactgaggcatggaggcaagaaggggctaacgcatgctcagggccgtggaactagtcctggcctgcagcaggactgacatcgcctggggccagcatggaacgcagcgtgaggtgggcaggggcagatccgagggctgcctctcccagggaccctgacaggtgccctcccgcccgcgcccgagacccttccccagagctgg

SEQ ID NO: 10871 - RNA, 7551 nt, Homo sapiens
  source 1..7551: mol_type = other RNA
ctgaatagctgggactacaggtacccaccaccacgcccagctaatttttttttttcgtatttttagtagagatggggtttcactgtgttagccacgttggtctcgatctcctgaccttgtgatccgcccgcctcagcctcccaaagtgctgggattacaggcgtgagccactgcgcccggccctaatttttgtatttttagtagagttgaggtttcaccatgttggtcaggctggtctcaaacccctgacctcaagtgatccaccccgcccccgcttcggcctcccaaagcactgggattacagggatgagccacctcgctgggaccagaccttactttcttgacttggccacaagtctgtcctgctcagagctgctgaaagtggctctcctgttgtatgggcttgggtgtggtgtggtggccctttccctgtcccagctgccttcttcctgggcactgaaaacgatgctaccattgtttttttttttttttttgagacggagtctcgctctgtcgcccaggctggagtgcagtggcgggatctcggctcactgcaagctccgcctcccgggttcacaccattctcctgcctcagcctcccaagtagctgggactacaggcgcccgccactacgcccggctaattttttgtatttttagtagagacggggtttcaccgttttagccgggatggtcttgatctcctgacctcgtgatccgcccgcctcggcctcccaaagtgctgggattacaggcgtgagccaccgcgcccggccaaatgctaccattgttaagtgccaggcgtcccaccatgcgggtcttcactgcgtatccacgtagctgcaccacgcaggcattctttcctcccttttgcagatgatggcaccaaagttcaagactcgcccagggccaccaagacagtcctctagactttggtcttccctccttgcctcctcggcctggggtggtggcgcctcggtctgagaagggtcgaggtctgggtgctgctagtggccctggctcagtctcagagctgcccggagggggtgaggatggctaacttaaggagcacaggcagaggcttcctgctggcaggaagagggctgagctgcggaaggccacccaggtggagtgtgctgcacctccttcagtggccttcaggagctctgtcctcacccagggattggggtgagtcagggcatggggaaacaggctcacagagcccacctgctcaccctgaccaccccaccccaggggaccccaggctcctaactctcagaatcccacagtctgtattggcggaagacgggctggcacccttgagttaggcccccagtcgttggcacagataaggggagctgctgctgaaggagcccgacggctgattctgtggaggcttctcagagctcctggcaggagcccctcaccgcaggaggcccacaacccctcccagctgcatatcggctcacattcacgcggctgccacacaagtgcgtcggaaactccacttggctgaacgtgattgtgctgctgtctgggacagtcttatgcacgtgagcccaatactggatgtcccgccattttcagccctggggcctatggcaaagtgacgcccccctcggagtgcacggcaggcaaggaaggtttaaacggaagttctgaccaggacgatgctgggtgcaagaggggacggggatggagcaaaacagaaaggatccaccagggcctgcaaccacgtctttggccccggtgaggggtgggaccttgtgtataggtccaggcagcagcagctgcagacagaggcctagagggtttggagaaggccgaccacaaagacacgcctagaccccagagtctagtgaggagagggactgggggcagtgtttcggcagcagacccagacccagactcagacccaagcccccctcctcactgatcaaaaccccaagggcagggagcccttcctgctccttcccgccagagcctggaggatgaggggcagacgggaggcccggccactggtgcctgctcctttgatcagctgtagtcccttccccttcacagggcacttgtcttgctggttggggtcaccagggattgctcccccaagtacccatcagcctccagggcccaaatgattccatgcagtagctctctccccctcttctgagaaggctcttggctcccagaaacggaaaccatgcctgggcctgctccccttccttgggctgtgacccccctgccacagaggccccccccccgccacagaggtcccccctgccacagaggtccccctgccacagaggcctggtggcccctgagctgctgctccgagtggaatgtcctggtctagaggcccttggctgctccagtgtcttaagacccatatatgagtgctggctctgaccttgaacaagctcctccatcgctccaggcctcgtttttcaggtgtatatgatgatagtatctctaggcctcgtttttcagttgtaaagcagggatgatcatatgtgtttaactcccagattgttatcaagtcaaggacaacaataggaaaacatgtcacctgtcagctccacacaaggcaaagtaggatgggtgacccctgactagggggtgggagtgcagggggcacccgacccatctggccagccacagcctctgtaccctgctcgcattttcaggcctcaatccccaagcactgttggccctggactgtttccccccctcaattctgtttctcaatgcctgcttcttcccagtaagtgccacaccctgagggtgggtgggagagtgaggcagcactgcccactttggctgggactgggcactgctggggacagcacgggccacgtcttccccatctcaagactggctttttggctaggcattgtgactcacgcctgtaatctcagcactttgggaggctgaggtgggagaattgcttcagcccaggagttccagaccagcctgggcaaaatagcaagaattcatctttatgaaaaagaaaaaaaaaattagccaggcatggtggcacacacttatagtcccagatacttaggaggccgaggtgggaggatcccttgagcccatgagttggaggccgtggtgagctatcagttgcaccactgcactccagcctggatggcagagcaagaccccaactcaaaaaaaaaaaaaaaaaaaaaaaggcggccttttcccagctggcagcaccctggctagttagggtttctccgaatctgcaactcctgtgtgatggcgggtctcaaatgctggcagcagagtcaccggtcagcggcaagacctggagtctccatttggaaccagcacccgggagcctctgctgggggtgatcatggagccgcacgtggaggctggtggctctgatggttcgagccgttcctcggcagcacagcacacccgctcctgaggagccacggagctcatgagcgttggcaaagtgctgtcagtgctggctgtaaggaaacaggcttgacttttaactcagcctttcccaaacttgactataatactttcttgaaaatcagaataaccactaacatcacaaaacgagtgttctcaggagtgggcatgtttatctcgttctctttttttttttctttttgagacggagcctcgctctgttgcccaggctggagtgcaatggtgcgatctcgactcacggcaatctccgtctccccggttcaagcgattctcctgcctcaggctcccgagtagttgggattacaggcgcacgccaccacgcccgattaatgtttatttttagtacagacggggtttctccatgttggtcaggatggtctcgaactcctgacctcaggtgagcctcctgccttggcctcccaaagtgctgggattataggcgtgagccaccacgcccagtctttttttaaatatttgagtgaaataaagcctaggagatatgtgttccaggcgcccaagctgttaatgtggagcttgaatgtggcctggacctgccctttcctcttctcctttcatccccctccctgccgcccacatcctgaactgctctgagcctgcagaagaacccagcgggaatcttcagggttgtggaagggtgtagggatggaaagggaccaggattcgcctgtttggctgggaaaatcggtagaggagggtggctcacacttctaagatgtctgcacaagcccagtttgtttgggggttggggaggaaggtcttttcctggcccactgtccctcccgagtcagcagtcccccagagagacgaagagcagctgggcacggctggagctggtcggtggcagagaatcttgtcctgccttttcttctcaagctcaaaataggcacatgcagctattaactgatatgccagaaggggcatcccttacccggaggaaaatggatttattgctttataaaaaagaagtctaataaaactgaagagaaaataactaaaaatccaaacacaactcacccctctaagcacgcccaggaggtctcaagacacacttctgggggcagtcaaggtgggcgggttggtgggccaggcggacgggcctcccccgtcatcagctccagggccccacggagcccgccggcagggggtgctgtgggcctgtggccttggacaagctcctggccccacgccaggatggctcctgggcactggcccagctgcaggcctggcggctcccgcctggtcagtggggataagggctaactcctagagcccaccccgaccccacacacacctcggacccacccacgtccccaccccggcctggacctccacgtctgccggccacagcctttcgtccacctccacaaaagcagctgtgtgtatgtacggggtgccctggcggcggtcctcaaattcccttcaggtggcagacagaacgagggtgacagtgaaaacgtgtccgcggcattggccctcggggaggaggcgaggggtccacccagcccgctaaaccctctccagggcataagccaggtggggcttctccaccggcctccaacgggtgggcaggccctggacaggcgacagggggctggaattacaaaggaattagcaccgacaacaggaagcgggtccttccttcctcaggcagcctcaggctggccggggagggggtgggggccaggcgcgggcgagacagtgcaagcctttgtcctcaggcaggtacggctgtgggcatgcagccgaggggcaggtggcaggcaggggatggcagccccctctgctttggcaagaggcagaatccagacactggcgggagagcgcctgcctgccgggcgttcctggctcctgctgcaggcaccacagagaccccaggccccgggtccccggggggcggcagagcaaagtcagggcagcccctgcgttcggcaggagaaaacgcgcgtgtccggggccctctcccgtccttccaccacagagctccgaggcagggccccgggagggagcgtgaacgctggcacggagacggcgaaggtcctgggggtgcgtggggtactctggaggggcaggacaggggtcagtcactgaagcacaggcaggagaccgcagttccgaggcggcagccactacacgaaggcctcctggttggacgagccgttgattttgaggaagagtttgtcatcctcctgcctctgctgcagctgccgctccagctggcgccggtagcagatcaggtagagcgggaggcagaagcccagcaggctgagaaggagcagccccacgttcacccacagagggtctccctggagaggacccatcatggccagaaacagcggctgctgcagaagggcgaagagcgcgctgatcagagactgcagtcccgtgaggctgccgaactgggtggaggggtacacggcagcgtacaggcccccgacagcggagtggatgaatcctcgcacgattgtgtgcaggatgaaggagaggatctggagaggcaggttgggaatgaggcaggtcaccccaaagcccacgagcagcaggttggtgaaggcgaaggcccgcatggcattagtgatcttctggatctgccggtcccgcttcttctttttcttctcgccttggttggcgtctttctcctcgggctcctcggaggcgtcttcacactccttcagcctccagtccatgatgtagccaatgacgggggccgtcagcaggcacagcagctggagcacgccgaagatggaggtgtagaggccaactgtcttctggtcgccgctgaccaggaacttgaggatgttgttcatagcccccatgtagaagatgagccgcagctgcgtgacgcacatggtgaccaggctgagcagcaggatggggctgaacacgctgtgcatgaaggagggggccactgcggcatccggctggcacttcacctccaggtcgacggtggacaggcacagcttgtggccctcctgcagcgccacctgctccttggcactcctcatggagctgcccacactcaggcgccggcccaccgtggtcacctgcttgtagaactgcttccctgtgatcttgtggtcaaagcccagccagctgaacttgatcttcaccgagtagtccatgtcctccggccccgggaagggctcaaggggccagttaaagaagcagttgaggaaaaccagcccggagcagccggcccagaccacgaggacgacgatgaaggagacaccagcatcatagatgagcttgattcctggaaaggtgactgccgaggaggcgtaggacccaatcatcaaggcaataaacgtggaccgaaggtcgccgaacatgttgggcagtgttaatgaggtgaaggtcatacacatcccaccaaagccattcagagccagggcgatgaagatgagcacggagagagcgtttggtttacttgctccgtacgcaatcagcaagcaggaaaccgcgaagcaggcgctggctcggtacacaggtaggagtaaaagccctctgacttgagcatgatgagcagcgagccccagcccaggaggactgccgagaagaggaggttctccagcacggccgtgcaggccatccaccagcggcgccgatgggcagtggccagggtgggcgccatggtgcggcgcggcgcggctccggctccggctccggctctgcaccacctttctccgcccgtgttcacgcactgctcggtcctccggggaccctccacccttgatcgtcatctgggtgctccctgcccgcgctggccaccttcaccccgttccccgtccctttcagggaaggtcccctctgcagggcgatgctacgggccacgtccgccagctggtacaagctagggagggttcgagggggctccgggtccccgtctgataagcccgggctccgaaagctcagctccccgtcttcgtcccccggattcgaggcactaacccgacccgggaagaccctctgactgccccagaatcgccttggtcaccctggctcgctccggggggctggcttagcaccccagggctgccgcgcggtgtccacgtctggaatcccagcggtttgggaggctaaggtcgga

SEQ ID NO: 10872 - RNA, 1824 nt, Homo sapiens
  source 1..1824: mol_type = other RNA
ctgaatagctgggactacaggtacccaccaccatgcccggctaatttttgtatttttagtagagacggggtttcaccgtgttagccaggatggtctcgatctcctgacttcgtgatctgcccgcctcagcctcccaaagtgctgggattacaggcgtgagccaccgcgcccggccgggttttacatctttaaagaagggggtctgcctgggcacagtggcttatgcctgtaatcccagcactttgagagaccaaggcgggtggagtacctgaggtcaggagtttgagaccagcctgacaacatggtgaaaccccgtctctactaaaaaaacacaaaaattagccgggcatggtggtgggcgcctgtaatcccaactaattaggatgctgaggcaggagaatcgcttgaacccaggaggtggacgttgcagtgagctgagatggcgccattgccctccagcttgtgtgacagagggaaactcctcaaaaaacaaaaaaccaaaacaaaacaaaataaaaaacaagggcgtctggctgtgttgccctggctggactggactccaactcctgggctcaagagatcctcccatttcagcctctggagtagctgctactataggttcgcattactaagtcaggtcgtttttacatttttaaatggttacaaaggtcatataaatacccacataataatatcctccattttatcctcttaaaccgcaaaggttacattatttattatctggccgcttaaaaaaaaattgggggcccctttctattccttcccagacctcagccaggaaacaaagcgccaagtaccggacctaaacaagcgctcagtcctgagaaccatgactccgccgtggccctggagcctggggctggctcccagctcgccgtccagccctccctggaggcagcgggttttcctctttcccgggggccaggctgagcgccccaggtggggctgtctgtgcccgagatgcccccaggcccctttcagagcgcccctgcggctcgggcggcggctcggcgcgggcagccccagcgatcgcgcaggcagaagtgccacaccagggcggcacagcttagcagggccagggccgtgcccaccccgacggccgcgtggaccagagtgcgggggttgggcggcaccgcaaggcggctgcaaggcccgaaggcagggatgtcggccccctcgaggccctctcctccagcctggggcacgcggcttgccccggcctcgttagcggccactacgcaaacgacataaatgccccctggcttcagccccttcagttcggctctgcggaccgtagcgttcagcgggggccccttctgcgcagcctcgctgccgtcccaaagcagcagccagtagtggaggaccggggagaagggggcacaccagtggaccactgcgcggccctcttcggccgcaatgcgcacttctcccatgcgcggcgggtcgggcggctgggcggggctggagagtcctgggcacaggcaggccgccggcccgaccctctgtagctccttgcagggcacctgcaggtgtcggcagtggtcgtagtcgcaggggacagccggcaaaggcggccacgccgtctcagtctcatctgcctcctcttcttcaaagtcttgaggggccaagggctgagctctgggaaccaagaaggtcacggccaggagccacagaaggcagggagagcccagcatggagacagtgggtaggccttgatgcagcgggaatccaccagctgacgtctgtgggtgttaggctgagggatccccaagatctcaggctgtgctgtcaggttgtatcttc

SEQ ID NO: 10873 - RNA, 1216 nt, Homo sapiens
  source 1..1216: mol_type = other RNA
ctgaatagctgggactacaggtacccacgaccacacctggctaattttttgtatttttagtagagtcggggtttcactgtgttagtcaggctggtctcaaactcccgaccttgtgatccactcgcctcagcctcccaaagtgctgggattacagccgtgagccaccatgcctggccctattgccttcctttaaagtgttgatcacagtaggaattaacctgttaagggactttgaataatccagtgattagggcttgaactaagtcatattataaagctgggaaagaggatagagaaaagaaatgatgtgggggcagaacctactgagtgtggggagtgattgcaaatgtgattggacaccatagaaattgttcagggagattccaaggttgctggcttgaatcgcaggtagtatgggctccacagaactcactcaggctcaaattgttctacatatttaatgaaactggtaccaaaatttcagctggcacttgttgcagaaattgagaaacagctctttgcaatcatctggaaatgcaagaaacccacaacagccaaaacaaccagcctgagagcatgactaactattattttttggcagtttgctttccaaatggttcactgtgattttcatggtgacttcttcgtcaatcaaattcagcaaacacaatctgccattttctcctcagtatttcctctcttcttgtgaattttcatgccagacacaagcggcagctccacaagcgggggtgttgcatcctctaccatttgcatgtgcaatctggaccaaggttagaaagctaattaaaatctctcctggggccatgcagcagaggaaaatggaggcataaagttctgcgtctggaaagttcaaggttgagggactggcatctactgatggccttcttactgcgtcatcccatggtggaaggtggaagtggaagagagccagcatgcctgggcgagccgttggtgatcaaggacacttcctgattaagacttgcttttagaacttcataactgctgtcgggcgcggtggctcgcgcctgtaatcccagcactttgggaggccgaggtcaggatcacgaggtcaggagatcaagactttcctggctaacacagtgaaaccccgtctctactgaaaacacagaaaatgagccgggcatcatggcgggcgcctgtagttccagctactcgggaggctgaggcaggagaa

SEQ ID NO: 10874 - RNA, 3226 nt, Homo sapiens
  source 1..3226: mol_type = other RNA
ctgaatagctgggactacaggtaccccaccaccacacccggctaattttttgtatttttagtagagacggggtttcactgtgttagccaggatggtctccatctcctgaccttgtgatccacccacctcggcctcccaaagtgctgggattacaggcgtgagccaccgcgctcggcccattattgttaatgatgctcaaactctccccattgggagccactccatgttgtctcctgcatccttttcaatgtgaccctcaccttccttgctatcaaggaagcaaggaatgaccagatgttccaggctcatcttgaattttttttcttgcctcagacctggaattggttatttcttcatgccctcatttctagtcggaagtggcgtttagacaccataacctgggtgctggggtgttcactgctattggatggctcattatttctaaactttatggttgacagagctagcaaacacctgctttactttgtaagacaaaaatatagcatgaattcatactgatgcttccaattccaattcggggctacgggtttttcaccttgtctctgtgatcttacgtgggcatctcctttcttccatgatcatgtgacaaagcctgtttggaaaagcaaagctccctactgtgattctcatcaagctggaagcgtgtgagaaagcacttcagtttcttccctcggatatgaacctgagctctctgatgaggtggtttagaagtggccctgggagaagcccacttcttggtcacaagatactgcattctcctggcagatgaaccagctgcttccagcatcctctgtgtgggtcctcacgcctagctgctctacgtgctggctgcacagtggcatcacatggggaagtagaaaaacctctgatgcctgtccccacccggcttaatcacagtgaagtcagattatctgggcctgggaccctaccatcattttttttaaagaattgcaggggccaggcgtggcggctcagagcttctagcactttgggaaaaagctcacagcttccagcactttgggaagccgaggtggtaggatcaggaggtcaggagattgagaccatcctggctaacatggtgaaaccccgtctctactaaaaatacaaaaaattagctgggcgtggtggcaggcgcctgtagtcccagctactcgggaggctgaagcaggagaatgacatgaacccgggatgtagagcttgcagtgagctgagatcgcgccactgcactccagcctgggagacagcgagactccatctcaaaaaaaaagaattgtaggtaggccgggtgcggtggctcatgcttgtaatcccaacactttgggaggtcaaggagggtggatcacctgacgtcaggagttcgagaccagcctggccaacatggcgaaaccccatctctactaaagatacaaaaattagctgggcgttgtggtgtgtgcctataatcccggctacttggaaggctgaggcaggagaattgcttgaacctgggaggtggaggttgcagtgagccaatatcacaccactgcactccagcctgggttacagagtgagactccgtctcaaaaaaaaaaagaattgcaggtaattctaatgtgtagccaggggatacagtcactgctctgttccttgcttctcagcagagggaagaaaaagaagcaacaaggctggcagatgaactctgccttcaaagcccattagcttcggcttgaattctggcactgccaggttctagctatgaaatctgaacctggctgggcgtggtggctcacacctgtaatcccaacactttgagaggctgaggcaggtggatcccctgaggtcaggagttcgagaccagcctggccagtgaaaccccatctctattaaaaatacaaaaattagctgggcgtggtggcatgcacctgtagtcccagctactcaggaggctggggcaggagaatcacttgaacccaggaggcggaggttgcagtgagccgagattgcaccactgcactccaacctggacaatagagcgagactccatctcaaaaaaaaaaaaaaaaaggaaatctaagtcagtgctgaccaatagcacttgtgcaaccttcaaatggtctatatctgcactgtccaatgtggtagccatcagccacagtacacggggctgctgggcacttgaactcattgttagtgcaacctagggtgtaaatgttaaaatttatttaattttaactaatttacacatcaatagccacaaggagccatcacagctactgtcttggacagcaccactctagaaaatgacctaacgtctcgtggcttcacatctgtaaaatagggaataataggggttatttcactggatattgacaggattagtgtcaggattagaaacaatgtatataaagttcctggttcccacaaaacactcaataaaatgctgcttatttattaacatcagcctaatactcaaaaaaaattgcctggaaaacaaatgttcagaagcaccctaccacagaggctaaaaattcagagccgttccagagaaactcagaaaatattccttaattgtagaagttcaatggcagcaggaggttatcagttacaagggctgtatttcattacagatccagccgcagctcaataaattaagcaatcactcagaataacatgttgctttaatcccctctcttggagcggttccaagttgtttggttttatacacgctcagccctgaaaggggactcatactgggctcatttctttcccctcaattcatcagcccctctctggaaacatctttgcatctcccaaccagcaggagagaggattccaagccaagcaggcctccttttatcaaaactggagccttttccatcctctggccttgacgtgttccacgtttcatttgctgaaattactggcaggtttatcgccgctgccgcctccgggggtgcacgggcccccccacccagggctgcgccttcccgggctccgggcaggcgtgcgccgggcggggggcgccccgcgggccctgcagcctccgcctcgattggagcccagccttaaatcctccaccgtggagaagaagggtacttccagaaaaaaaatccgcccctccccagacgagatccaagtgatgggcggggagcgtagaaaatccttttctgcagagagcgcgcagccgacggggctgcacccggcctccacggtccgctgccgccac

SEQ ID NO: 10875 - RNA, 3084 nt, Homo sapiens
  source 1..3084: mol_type = other RNA
ctgaatagctgggactacaggtaccccaccaccacacccggctaattttttgtatttttagtagagacggggtttcactgtgttagccaggatggtctccatctcctgaccttgtgatccacccacctcggcctcccaaagtgctgggattacaggcgtgagccaccgcgctcggcccattattgttaatgatgctcaaactctccccattgggagccactccatgttgtctcctgcatccttttcaatgtgaccctcaccttccttgctatcaaggaagcaaggaatgaccagatgttccaggctcatcttgaattttttttcttgcctcagacctggaattggttatttcttcatgccctcatttctagtcggaagtggcgtttagacaccataacctgggtgctggggtgttcactgctattggatggctcattatttctaaactttatggttgacagagctagcaaacacctgctttactttgtaagacaaaaatatagcatgaattcatactgatgcttccaattccaattcggggctacgggtttttcaccttgtctctgtgatcttacgtgggcatctcctttcttccatgatcatgtgacaaagcctgtttggaaaagcaaagctccctactgtgattctcatcaagctggaagcgtgtgagaaagcacttcagtttcttccctcggatatgaacctgagctctctgatgaggtggtttagaagtggccctgggagaagcccacttcttggtcacaagatactgcattctcctggcagatgaaccagctgcttccagcatcctctgtgtgggtcctcacgcctagctgctctacgtgctggctgcacagtggcatcacatggggaagtagaaaaacctctgatgcctgtccccacccggcttaatcacagtgaagtcagattatctgggcctgggaccctaccatcattttttttaaagaattgcaggggccaggcgtggcggctcagagcttctagcactttgggaaaaagctcacagcttccagcactttgggaagccgaggtggtaggatcaggaggtcaggagattgagaccatcctggctaacatggtgaaaccccgtctctactaaaaatacaaaaaattagctgggcgtggtggcaggcgcctgtagtcccagctactcgggaggctgaagcaggagaatgacatgaacccgggatgtagagcttgcagtgagctgagatcgcgccactgcactccagcctgggagacagcgagactccatctcaaaaaaaaagaattgtaggtaggccgggtgcggtggctcatgcttgtaatcccaacactttgggaggtcaaggagggtggatcacctgacgtcaggagttcgagaccagcctggccaacatggcgaaaccccatctctactaaagatacaaaaattagctgggcgttgtggtgtgtgcctataatcccggctacttggaaggctgaggcaggagaattgcttgaacctgggaggtggaggttgcagtgagccaatatcacaccactgcactccagcctgggttacagagtgagactccgtctcaaaaaaaaaaagaattgcaggtaattctaatgtgtagccaggggatacagtcactgctctgttccttgcttctcagcagagggaagaaaaagaagcaacaaggctggcagatgaactctgccttcaaagcccattagcttcggcttgaattctggcactgccaggttctagctatgaaatctgaacctggctgggcgtggtggctcacacctgtaatcccaacactttgagaggctgaggcaggtggatcccctgaggtcaggagttcgagaccagcctggccagtgaaaccccatctctattaaaaatacaaaaattagctgggcgtggtggcatgcacctgtagtcccagctactcaggaggctggggcaggagaatcacttgaacccaggaggcggaggttgcagtgagccgagattgcaccactgcactccaacctggacaatagagcgagactccatctcaaaaaaaaaaaaaaaaaggaaatctaagtcagtgctgaccaatagcacttgtgcaaccttcaaatggtctatatctgcactgtccaatgtggtagccatcagccacagtacacggggctgctgggcacttgaactcattgttagtgcaacctagggtgtaaatgttaaaatttatttaattttaactaatttacacatcaatagccacaaggagccatcacagctactgtcttggacagcaccactctagaaaatgacctaacgtctcgtggcttcacatctgtaaaatagggaataataggggttatttcactggatattgacaggattagtgtcaggattagaaacaatgtatataaagttcctggttcccacaaaacactcaataaaatgctgcttatttattaacatcagcctaatactcaaaaaaaattgcctggaaaacaaatgttcagaagcaccctaccacagaggctaaaaattcagagccgttccagagaaactcagaaaatattccttaattgtagaagttcaatggcagcaggaggttatcagttacaagggctgtatttcattacagatccagccgcagctcaataaattaagcaatcactcagaataacatgttgctttaatcccctctcttggagcggttccaagttgtttggttttatacacgctcagccctgaaaggggactcatactgggctcatttctttcccctcaattcatcagcccctctctggaaacatctttgcatctcccaaccagcaggagagaggattccaagccaagcaggcctccttttatcaaaactggagccttttccatcctctggccttgacgtgttccacgtttcatttgctgaaattactggcaggtttatctcctctggaatggctggagtcccctggatcccccagggttgaaattgcacagacacactgtgttcccaagaactcccccaaataccaacccagcttcgggccagaaaataaagttgtgcttcctcctccccagtccaatgtcactttgtt

SEQ ID NO: 10876 - RNA, 3287 nt, Homo sapiens
  source 1..3287: mol_type = other RNA
ctgaatagctgggactacaggtaccccaccaccacacccggctaattttttgtatttttagtagagacggggtttcactgtgttagccaggatggtctccatctcctgaccttgtgatccacccacctcggcctcccaaagtgctgggattacaggcgtgagccaccgcgctcggcccattattgttaatgatgctcaaactctccccattgggagccactccatgttgtctcctgcatccttttcaatgtgaccctcaccttccttgctatcaaggaagcaaggaatgaccagatgttccaggctcatcttgaattttttttcttgcctcagacctggaattggttatttcttcatgccctcatttctagtcggaagtggcgtttagacaccataacctgggtgctggggtgttcactgctattggatggctcattatttctaaactttatggttgacagagctagcaaacacctgctttactttgtaagacaaaaatatagcatgaattcatactgatgcttccaattccaattcggggctacgggtttttcaccttgtctctgtgatcttacgtgggcatctcctttcttccatgatcatgtgacaaagcctgtttggaaaagcaaagctccctactgtgattctcatcaagctggaagcgtgtgagaaagcacttcagtttcttccctcggatatgaacctgagctctctgatgaggtggtttagaagtggccctgggagaagcccacttcttggtcacaagatactgcattctcctggcagatgaaccagctgcttccagcatcctctgtgtgggtcctcacgcctagctgctctacgtgctggctgcacagtggcatcacatggggaagtagaaaaacctctgatgcctgtccccacccggcttaatcacagtgaagtcagattatctgggcctgggaccctaccatcattttttttaaagaattgcaggggccaggcgtggcggctcagagcttctagcactttgggaaaaagctcacagcttccagcactttgggaagccgaggtggtaggatcaggaggtcaggagattgagaccatcctggctaacatggtgaaaccccgtctctactaaaaatacaaaaaattagctgggcgtggtggcaggcgcctgtagtcccagctactcgggaggctgaagcaggagaatgacatgaacccgggatgtagagcttgcagtgagctgagatcgcgccactgcactccagcctgggagacagcgagactccatctcaaaaaaaaagaattgtaggtaggccgggtgcggtggctcatgcttgtaatcccaacactttgggaggtcaaggagggtggatcacctgacgtcaggagttcgagaccagcctggccaacatggcgaaaccccatctctactaaagatacaaaaattagctgggcgttgtggtgtgtgcctataatcccggctacttggaaggctgaggcaggagaattgcttgaacctgggaggtggaggttgcagtgagccaatatcacaccactgcactccagcctgggttacagagtgagactccgtctcaaaaaaaaaaagaattgcaggtaattctaatgtgtagccaggggatacagtcactgctctgttccttgcttctcagcagagggaagaaaaagaagcaacaaggctggcagatgaactctgccttcaaagcccattagcttcggcttgaattctggcactgccaggttctagctatgaaatctgaacctggctgggcgtggtggctcacacctgtaatcccaacactttgagaggctgaggcaggtggatcccctgaggtcaggagttcgagaccagcctggccagtgaaaccccatctctattaaaaatacaaaaattagctgggcgtggtggcatgcacctgtagtcccagctactcaggaggctggggcaggagaatcacttgaacccaggaggcggaggttgcagtgagccgagattgcaccactgcactccaacctggacaatagagcgagactccatctcaaaaaaaaaaaaaaaaaggaaatctaagtcagtgctgaccaatagcacttgtgcaaccttcaaatggtctatatctgcactgtccaatgtggtagccatcagccacagtacacggggctgctgggcacttgaactcattgttagtgcaacctagggtgtaaatgttaaaatttatttaattttaactaatttacacatcaatagccacaaggagccatcacagctactgtcttggacagcaccactctagaaaatgacctaacgtctcgtggcttcacatctgtaaaatagggaataataggggttatttcactggatattgacaggattagtgtcaggattagaaacaatgtatataaagttcctggttcccacaaaacactcaataaaatgctgcttatttattaacatcagcctaatactcaaaaaaaattgcctggaaaacaaatgttcagaagcaccctaccacagaggctaaaaattcagagccgttccagagaaactcagaaaatattccttaattgtagaagttcaatggcagcaggaggttatcagttacaagggctgtatttcattacagatccagccgcagctcaataaattaagcaatcactcagaataacatgttgctttaatcccctctcttggagcggttccaagttgtttggttttatacacgctcagccctgaaaggggactcatactgggctcatttctttcccctcaattcatcagcccctctctggaaacatctttgcatctcccaaccagcaggagagaggattccaagccaagcaggcctccttttatcaaaactggagccttttccatcctctggccttgacgtgttccacgtttcatttgctgaaattactggcaggtttatctgccgcgatccctgccttggctggcggaaggtgccaggcgggaagaaggggagcactcaccgccgctgccgcctccgggggtgcacgggcccccccacccagggctgcgccttcccgggctccgggcaggcgtgcgccgggcggggggcgccccgcgggccctgcagcctccgcctcgattggagcccagccttaaatcctccaccgtggagaagaagggtacttccagaaaaaaaatccgcccctccccagacgagatccaagtgatgggcggggagcgtagaaaatccttttctgcagagagcgcgcagccgacggggctgcacccggcctccacggtccgctgccgccac

SEQ ID NO: 10877 - RNA, 2876 nt, Homo sapiens
  source 1..2876: mol_type = other RNA
ctgaatagctgggactacaggtacccgccaccacgcccggctaatttttttgtatttttagtagagacggggtttcaccgtgttagccaggatggtctcaatttcctgacctcatgatccacctgcctcggcctcccaaagtgctgggattacaggcgtgagccaccgtgcccggccaagaccccttcttaaaaacgtactcgagtatgaagttttgtgaatccaattttagttttaccaaagaaattgtaccataatacactccttgccctcaactgcatgcccattagaaatgagcatgaacactttctggaattaacaatacatcacatattcatgtgtcgaaagtattgccatgtgtagaaagtgtttacaagtcaaatgggataacagagtaaaccaggcacatcaacttgtatgaatgtgatacagtagcactgttcactgtgtaagatgctgcatttttctttaaacttttggaatgatttgtactcccaacaatccacactagagagagttagccccatcagaagttcagagggtttgagttcctttttgagtggtaatctagaacactttttttagtcaggaaatattttcccataaggatttttctaattgagatgtcatttacatagtataacattcactctgttaaaaatatatggttcaggccaggcacagtggctcacgcccgtaatcccaacactctgggaggctgaggccagtgatcacctgaggtcaggaggtcgagaccagcctggccaacatggtgaaaccccatctctactaaaaatacaaaaattagacaggtgcctataatcccagctactagggaggtggaggctgaagcaggagaatcgcttgaatctgggaggcagagggtgcagtgagccgagactgagccactgcaccccagcctgggcaacagagtgagaccctgtctccaaagaaaaagaaaaaaaaaagtgtatgggtgagtgaattttagtatattcacaaagttgtgcgaccatccccagacataactcccaaaccccacatccatcacccatcagtgataacttcccacttttccctccccagcccctggcagccactattctgctttctgcctgcctgggtttgcctgttctagccattttctatcaatggaatcatagaccgtgtggcctttgtggctggcttctttcactcagcatgacattttcaaggttcatccatggggtgctgtggaccagcactctgtgcctgtctgtggctggaaatattccaggacttggtgttacgggctgagcttgagttgtgacctcttcaaactccaatgttgaagtcctaaccctcagaaactcagaatctgactgtgtttggagacaggcaaagaggtaattaaattgaaatcaggtcactagggtgggccctcatcccatctgcctagtgtccttgtgggaggagatgaggacacacacactgagggacaaccacatgaggacccaatgagaagaggccatctgcaaggcaaggagagaggccttagaaggaaccagctccaccaacatcttgatcttggacttccagcctccagaacttcttgaaaattgttttcaattattgtactccatttgtggaactcgtgtcggagtctggtaaacagccgaatgtcttcctcccctacagtttcctctccttgcatgagagcagtgatgtcctgattaaaggcattaactttatctatcaggaagaacattttttcattttcgtcttccggtatgtcgacaccatacttttgtagctcctctgttattctctggtgagtctccttgatttgattttctaacaggggcagagatttacagatatgtgtgatgagctcgctggtaagtttttctgccaggcagggaaccgtggcctttccttcctccagcagatccctgaaatatgggtggttctcaaagaagatcttctctctctgcagggcttcggacaggctcagctggtcctggatctcctgctggccccggcacttgacaatcatgtaacccttcttcaggtggaacacgaggttccgcaccacgtccacaaccttgtcttcagttcctttgtccaccagatcaggcttcgtcaagattccgatggtcctgtctccctcggggtccacctcctgggccatgctgagagcctctgtggtggcgatgtccacattactggggaccaccaccaggctgattgtctcctgcctctggatgtacttcttgatgagtgtcttgatcttatacccaatgtcagcaggctgattgcccacagccactctggttatgccaggaaggtctattagagtcagatccgggacatctcgggagctgatctccagggtgattagctcatgactgattcccattccttccccggcgatggcattctgggctttattaatttccttttctacctctgaagcatccgaaatctcaatctcgtagtcctggtaactgaccttgcctctccacttatcttcgttcacaagtttcttcagtttcagcaccagcgggcatctggtcacgatcccgctgcctctgggaagggcaactcctgacagtgcctccaacacggagctcttgcccgagctctggtccccgatgacggcgatggctggcagggccaggtcctgctccacacctagagcccgcagggagtcaatgaggtcgatgcaggggcgcaccttctcctcatactggctgcacaggttgttctcagccaccgagcctggatttttctgggccacagtagcatctccattcagtaatagagggtgggatgcagcagctggatcagcttttgcgatgtccacttcggaaacaaccatcttccttctttgcaaa

SEQ ID NO: 10878 - RNA, 4659 nt, Homo sapiens
  source 1..4659: mol_type = other RNA
ctgaatagctgggactacaggtacctaacaccacacttggccatctcaaggacattttatgacaaagaggagagtgctgtgcacacagaaggagctcaaccaatgttggttagattggaagaaatggtgctccctgcccccagcccctcaccgtgatggcgtctatcttgaagagggctttggcctgggtgctggtgtaggcgttgaagcggtacgtgatttggttgaggttgtcgatggagtaggcctggacccgcacaatctcagtacccagtgccagattctccaggatggcagcctcgtatgaggcattggagaactgcacggcctcgtccagctcgttgagcagagtgatgtagacgctgcagaagccctggttgaagggcggggcctggtcagtggccgacacattcatcatgtagctggtcttggtctcgtagtccaggtaattcacggtgatgataagccctgtgctctcgtcaatctcaaacttcccctctgcgcccgacaggatgcggtagttcaccaggccaccatccccagagtctcggtctgtggcttggaccacgatgactgacgttccaatgcctgcggtctctcgaagccccagacggctgtactgctgctgtgtgaacacgggggcctcatcgttgatgtcctccacgtacacaatcaccctgacggagctccgcatggggcccaggtcgtggttgtaggcctccactatcagcacgtgggatgagttccgctcccggtccaggggccggggccctcgcatcaggagcccattgctgacatggatccggaagttgttgccatggttaccatggaggatgcggtaccacacacgcccaaactcgccctcatctgcgtccgtggctttcagctgcaagatgctgtggccttcagggatgtcctcagggacgctggcctcatagctgctctgcagaaagatgggccggttgtcattcacatccaggacagtgacgaacacggtggctgtgcccgtgtgtcgcttccctacagggccgttgtcgatggcctccaggatgagcatgtaggcggctgtggtctcccggtccaggcccaccacggttctcacaacggcatcgcggtaacccacgctgaacttcccatccacgttgccacctgtgatgaagtagctgagctctgcattgaggcccacgtcgttgtccgtgcagttcagccagaccacccggaactcgcgtggcacgtcctcggacacagacacattgtacacggccgggaagaaggtgggcgtctcgtcgttcacatccagcacatggatggtgagcgtgctggtggagctcttggtgggcgtgcctgcatcactggccaccacccgcagctggtactccgcgatgcgctcgcggtccagctcggtggtggtgaccaccacgccgctgctgctgttgatgaggaagtccatgcggggcatgcccaccggcatgcggtaggacaccaggccgttcaggccctcatcgaggtcgatggccaccacttggtagatggagacccccgccgggatgccttcaagcacctcggccacaaaaggcaggttctgaaaggtggggtcattgtcattgagatccaagaggttcacaaacactgtggcactgctggtggctttcagagggggcctgccacagtcagtaacagagacgacgattttgcgcatcagctcggcctcatgggggtcggggttctcccggtccagcatggcgtgggtggtgcggatcttgcccgtggtgctgttgaggctgtagaacttgttgggtggctggatgctgtacaccagggtgccattctcccccaggtctgggtcaacagccaccaccgtggtcacatcagagtctggaggggtcatctccaccaggttgatgtagtagggtgcgtccttccacgtggggtggttgtcattgatgtccaggagggtgatgtttacggtggcgatgccagttttctggttgtggcccacacccccgtccactgcgcgaacgatgaggatgtattcagacttggtctctcggtcaagcagagacgtggtggtgatttcccctgagcgggcattgatccgaaactgggtggagccttccaaggagtagatgatggactcctggccgtactcccgggagcggtccaggtctgtggcattcaggaacagcaccgtggctcctgccatgatgttctccaccacggagacgaagtaggcgggcttgctgaaggtgggagggttgtcattctcatcaaacacctcgatggtgacagggacggtgctgttgagaggggggttgccagcatccatggccatgaccgtcagataaatcagcccattggatatctgttcataatccagggggcgactgacgctgatcactccatagccctcgtacaggctgatgtcgaagtagctgccaaaggcagatgcactgacaatgctgtaggtgatctggttgttgggaggggagtcttcatctgttgcccggagccgcaccagctgtgtgacagaaggctcgttctcccgcagagcacccacgtaggcatccttctggaaggtgggcacgttgtcgttgacatccaacacattgatcctgacccggcctgtggtctcctcgccgcccccgtcccgggcaatgatcgtcagggtgaagcgctggatgagctcatagtccagcctggcaatcagcatgatgagtcccgtgtccttgtccagcgagaacctgtcagggtcatcactgaagaagtagctgacttccccaaaggtgcctgcatcattgtcagttgccaggactgtcagcacagaggtccccacggtgacgttctcgtacaggctgatgttgtacagtggctggctgaagatgggccggttgtcattttcattgatgagagtgatcttcaccttggcatagcccacatggtcaggcacactctcattggcaaagagatcaaagtcgtagcggtccacggtctcgtagtccagtgggatggccacccgaatacgaatgtccgccttcccctggacggaggtcggggagatgatgaagtggtgggagttgttccccaccaagtacacctcaaacatgctgttcaggcccaaattctcatccttgtccaccacctggatgaagagtggaagggcaaagccgacctgtgccagctcagtgatggccacgctgtactcggagctgttgaactccggggcattgtcattgatgtcaataaccaggatattgaaggtcgtggtgactgtagcgtcagatggggtgcggtcatcgttcagctccgtgcccttcacagtcaggatgaagccatggctgtacagggggttctcccggtccagcaggccattcaaggtcagcactccgctgatgtagtccagggcaaagatgctgttggtattccctgaaacgatggtgtagccaatgccccggggacgtcctttatcctggtctatggcggtgatgatgcgcaccgtcgtgcccggaggagaatgctcgtagatgttggtgctgtaaggcaggttgatgaagatggggtccatgtcctggacatctgtgatgatgatggccaagttggccagggtggacagaggcctggtcttgtcttgatctgtggcgttgaccgtgagctggtaggcctgtgtggtctcgtagtccagctcccggatcactgtgacgataccgcgggcgctgtcaatggcgaagaattgggaggggggctggaaggagtagaggacgctgccccctgcccccaagtcggggtctgtggcattcacgatgaagatgggcgtccccactggtgtattctcagggatgcggacgctgtagggctgattgtgaaatgtgggcgcgttgtcattcacatccccaacctggatgttcaccttccgtgtgatcaccccctggtggtcgctgacagagaactccacggtgaactctgacttggtctctctgtccagtggctgccggagccacaccacgccagtgtcaggctccactgcaaagaagcgagaggcctcctccccagacacgccaaacaccagggggtcattgtccatgtcttgggccagcaactgggtcacagaagaacccacaggcgtgtcctcgctgatcagcaggtatgtatcaaagaagtggttggtgaagaagggcagccggttcacctggccccagcatccagagatcagcaccaaaagccaggccacgtggcagctggtggcaacatggcgccccatggctccgtgtgcgtgtgtgcagcggcgccgcgcctcgcctcgcctcgggctctgctctccgccggatcggcccccgcgggccgcctgctctggccctggccaccgccgcgtcttcccgccggcgcgaaggctcatccgcggcgtgccggcagctcctgggtctccgcgggccgctcgccgctcgccgctcgccgctcgcaacttcaggcgcgccgggggctcggactgggcgcgccccaaacgtccagaggctctgccaccccgcgctccatgcccaggccgggctgactagccccgaccacctcagcgtccggccgccgtcggacgcgtcctctagccaagcatcgcgcctgcagcccgcgtccctctctcccgagccgccgccgccgctcaagtccgcgatc

SEQ ID NO: 10879 - RNA, 3608 nt, Homo sapiens
  source 1..3608: mol_type = other RNA
ctgaatagctgggactacaggtacgtgccactatgcccagctaatttttttatttttatttttagtagagacggagtttcactatgttggccaggctggtctcaaactgacctcatgatctgcccacctcggcctcccaaagtgctgggattacaggcatgaaccatcgcacctggcccaaaatgtatttatttttttaaggtacacattgaaatgagaagttttaaaataattatctctcttgaaaatatgagctttatttatctcataaataagcttcagatttgagggtaacattctggatctcggtccaagcactgcttcttgccctatagccagaatcttctcatccagtgacaagggcagggccagataatccatggtacacagaccctgattctaaaattcagtgagtccgatgctagcttccactgtctgctttttagttagagaattcctgactttttctattatgtttattacctaaaggtgaagtgttggattgcttgtttttttcctcccctactaagcaggttttcactccacttcccacatcccaccccagacctctcacaaaaagagtctcatctgatatgtgaatgcagcttatctccccataggtagccaggaacagggtgcacagtcaaggcaaccccaaaaatggcctctctcccggccgcgcctgcaaagtcgtcctgagcgtcctgaacgttcctcagctggaggggcttttccctactcagtgtctggaccattgccaagaagatctgtccagctgtaagcctgattttatatagttattttcacttattttttattttgcaaaatgtaaacgaatctgtttagctaggaaatcacgtcccttgaaagtgattataacctaatttgacatgcagtatttgtatacttattctagtgttatgatgcatttactgtgtttacataaatacagatttctgtataattaccacaagataatgtaaagagttaatcatatgaaatcccccaaaatctcatttgagtgattttttttttttaatttgaaagtaaattttcctttagaaacaaattgggcccatttccaaaatattctatacatcttctttgagaggctcacaaaaacatctactttatccattcttactgatcattaattgatatggtctaattgcccttacacctaatacgtgccaaatagcagcaaagatagcatagacatgagtcttgccttcaagggtgttacatgtaaacaagtctggaagggcttcatggggaaaggtggaactctgccttgaacttatcggctgatctttgataatcactatggttccttcatgatctatacaatgaaaactgaatgtaagaaaagatttttatagaagaaatatcaaaaagagaggcaactagcatgaaggaagaactatacagattttaaaacttacctctttttattttattgacaaatgaaagaatttccctcaaattggaatactttactaaaactgggaaggagtaatcacataaagaacaacccaatagttctatactcatacaccaactgaagctatactagtagatagcaatatacaagtatatcaatatactacttttttatctttctgaaggtaaatcagtgtttctctctgcacttatctgcttccattcattcagttttttgtttgtttttgtgacagagtcttgctctgttgttcagactggcatgcagtggcacaatctcggctcactgcaaactccccctcctgggttcaagtgattcttgtgtctcagcctccccagtagctgggattacaggcatttgccaccacacccggctgatttttgtattttcagtagagactgggtttcaccatgttgcctaggctggtctcaaactcctgacctcaagtgatctgcccaccccttagcctcccaaagtgctgggattacgggcatgagccactttgcccggcctcattctggttttgttgtgtgctttgttctgtcttggaatatttgagggttaagaaattaggtcaaaagtctgccagcgtacaccaagctgtgtgtatagtgaaaggagggctggcaaaatgtctaccacggcatctgctttagaaaggtgaagctatcactgcaggtgtacacatcactaatgccatcctttcttatcactgggtgctggaaactcaggtaaaccagggaggagaaagtatcttcatttctcccaagagtgttatttctccatcatcatgttcaaagccttctctcaattctttgagttcttctctttatcttgtttcctactgccaacacaacttgcttctgctgtggcacatcttgacaaatagtgcatcttcactttccagtctcttcagtgtacgcctttcttgataagccccatggtttccttcttggagaagggattgtgctctgtacagatgcattcagtcttcttgaagcctaaactctgcttggtggggccaggaaagaggaggcatgtttcagtgttctgcagaagaaagtcaagaatcctagccccttgctctgtgcctcagtttctgcatctcagggagcctcagtcctgtctgcttctttctttcattttgacttcctcggtcagcttttccctctgccagaagagttgacatagaactttctctcccacccaatgcattccagaggaactttaggatgcccttgggataagagtgtttagagaagaaaattttctttgaaatcatcatgaagtaattccaacgctctgtgtgagataatcatgcttccagccaacactttgtgcaggagaaagtcctcgaactggctccaaaacttttcaattcctgacaaatgcactggcccctctccaaggagctgggcagcaatctgtgctttatgctggtgtgtggtggtggcaataccactggtgggagagccaggaggcggaggcgttcttctcaagtaagaaagatctgaagaccagtggccttggggacgcacccaggcaccaagaactccaactcacggcaccaagaactccacggtagggggcaggttcttaactgctttcaattttcctgtaaagaagtatttagagttgataatttcgaaggtccctttcatcacttaattccaagcttaagataatcttttcaccattagtcagtagcctttggcagtgatagctctcttacttgcttcatatcctgccattcacattgcagctactctttggtgaagatctttttcaattattttggggagcttgttgttttttaatgtagggttcaagtcctgtagtgaaatctgtttcatatttgcaatcagttttcagctcctggaagaatcccaaattggtaagtcccttaagtgtcacatcctagcctggcagtcagatgttttcagcaaagcaatagtttcaaacgtcttctcatatggttcagtgtcggcgttgaacagattccatataaattgcagtgacttctaagacatcttcatttgtttcccttccccaacccacccctcctccactgaagtccttaaagtccccgacctgttccacatccacctgtttaaggcattttccactcatctcatttcagagacattct

SEQ ID NO: 10880 - RNA, 2755 nt, Homo sapiens
  source 1..2755: mol_type = other RNA
ctgaatagctgggactacaggtacgtgccatcatgcccagctaatttttgagtgaaagccagtgcacctggcccatttgttatgattaatgaaccaatattgagacacaagtaactgaagtccacactttgacagtttccttaggtttgcctcatgtccctaatgtggtatccatcagaacaccccattacattgagttatgtgtctttaggctccttctcagactttcctcgtttttgatgaccttgacagtttcgaagagtactgggcagatattttgaagaatgtccctcaattaaaatgtgtctattatctcctggttagactgggactgcaggttacagaaaggaagcatctaggggtgaagtgccactgtcaccccatcacatcagggacacacactgtcacctcgactataactgtgaggctgacctgcgtcacttggctgaggtggagtctgccagttttctccacaataaagtggctctttccctccttttctttattgcactctttgggaggaagtggctatgtgtggtctacacttaaggagaggggagttacgtttccctccttgagggtgagtatctacaaaatttatctgggcagcttttttttttttttttttttgagttagggtctcagtctgtcacccaggttggagtgcagtggttgcctggccttgacagctttttaatagtttaaaatgaattgaggctgggcgaggttgctcatgcctgtaactccagcactttgagaggccaaggcaggtggatcacttgagcccaggagttcaagaccagcctgggcaacacagtgagaccctgtgtctactaaaaatacaaaaattagctgggcatggtggtgtgcctgtaattccagctgctcaggaggctgacatggagaatcacctgagcccggggaagttgaggctgcaatgagcggtggtctcaccactgcactctagcctgtgtgacagactgagaccctgcctataaaaaagaaaagaaaaaagaactgaaataagacccaagtccaacattagcagaacctctctaggatgtccacagaaacgactctggggttctgaggaacacagtctaggcaaacctgggcacatcccctcagtcccacagttgtaaatgtattgtaacacgtaacagttgtgagattcaggcgcggtctgggtctctgttcctggaaagtgtgatcctgtgggtgcagcccctgctcgcttggctgtgttgcctgcctggcccctgctctaatgagcccactgcccagagtttgctcaaaccacccaattccgagtctgggaaccaggagaccgctggacaccccgctcaccacacagaagactgtggcctgagtcaggagaaggaagtttctggcggtcgagcttccacggcttcctgagggaggttgcagggagccgagatcgcgccattgcgctatagcctgggcgtcgcagcgagactgtctcaaaaaaagaaaaaaaattctgagcgagattccagggcttcctgagggcgcgtttaagttgcagttgctgaggaggctgcaaggtgagcttgcgtcagcgaggagccactccagcacgctcgggaagggcatcgttactgctgcaaacaagcacacggccctccacgacgaaccttttgcaagtgaaggcgcacgaacaggcccggaggactacaaagaaacccagaaaccagacttggacacatgaaataaaggggttagctgaaggaatactccacagttaaggacggcctgcgcgaggtcaccggccctgtcttggttttttgccacttcgctccagttagtttcccaagttccacctacgcgcgcgccagctgagaaaacgcccaccccggcggtcccgccacaggtcacaggcggtgcggaccccgggactgtgtccgggcttcggtgtccagagagctccaagacacccaaaccttccgtggtttccacctctgcaagcttatgttccgctgagctcaagctgagggacgacgacctcatgcgacgtcagtttccccctgggaccacgaacccacggccccatttctcttctgtctactaaaaaccttttcttttcttttttttttgagacctaagacatcagtgagacacacgagcagacacgggctcggtcgggaaaggcgggagctccaagcggcggggcctgcaggtccaggcggttcgcgggctttctgaccgcattcggccgagttcttctctgaagacccaggacccccggccgagggggcgcattcggcgggctggtggcgtaggattttgtttcgggttcccagggtcccggcaagggtgagggagcccttgcggatcccctgagatccacctcagcagcctcctccgtggtaggcctcaacttcccgcggcggcccacagccaacgactaatgcctgagcgggagaaaacggcctggccctgtccgggtggttgctgagcaccgttcggcgccgcccgcgcctgcagggagcccggcccgctgtcctggtggacacaaagcccaggggccgcccgcgcgggaccagcagcgcgaactttttgccgctcggccagcctggcaggggattttaaaatcggccaatcacagcgggcgccaggcctccgctttccgcttactggtcctgccgtaggaggcgggtacgtgagcgcaccaatctgtggccggcgagcgtaaagggcggggctccgcccaggctgcaccgcccagagcgcgcgt

SEQ ID NO: 10881 - RNA, 2242 nt, Homo sapiens
  source 1..2242: mol_type = other RNA
ctgaatagctgggactacaggtacgtgtcaccacatcgcgttaattttcaaatttttaggagagatgaggtctcactatgttgctcaggctggcctcaaactcttgacctcaagcgatccccccgtgttggccttccaaaatgctggaattacaggtgtgagccaccatgcctggcctaattttgcttacacacacacacacacacacacaagaaaattgcaatttcaggagccatgacttatgacatcattgattcctgatggggcagctcaaaaaaaacaaaacaaaacaggaccataagatggcagtattgcataacaagctttactgcacggcacttagataggtttgcatgcggggaatgtcccttccagcaggactccttccagaggaactcctgggacagaggagagttagaggcagggcttaagtgtctaggtgatgtcattgagtagcaaggtggggagagtctgcatcatagaactctgaaaggcaacaataatttggggtttcttatggctgtaagatttttcttctctgtgattaataggtgttgttgggtgcaattttatggggtatgcaaagcaggtgggctctaaatgactaaacatatgcttatttgtgcaatatttatagcaatggattgtgtgagaatttgagcttggtgctggtgggctttgagctgagaggtccctgcctgcctgctgtaaagaaataaatgagatagggctgatagaaagacactgtctttggctcacttatacagcaagtgacaaccaatttagttcagacctttcttgcttctagacctgcaccatccactcttatccacttctcattcttcctggaagctgccacggaacatgcagacccccgtatccacttttgccagtagggacacccacttttgaaaagccacggacccctggcaacgcagctgcagacataccatttaactcaccctgcctggaaaaggaaagtaaatgttttcttcccaatttttgctagggaaatccaggcacatatatgtattcagtaactcaatgatataaatttcagggcttgtgtctgtgtgttattggaaaagcatttgaggctggctgtcatggttcatggctgcaatctcaacactttggaggctgaggcaggaggctcacttgaggccaggagttccagaccaggctggacaactctacctctacaaaaaaataaaataataagccccgcatggtggtgcacacctgtagttctagctactcaggaggctgaggtgggaggattgcttgagcccaggaattcaaggctacactgagctatgatcacaccactgggcctgggcaatggagtgagattctgtctctaaaaaaaaaatgcatttgagaattttagcaaatctaagtacatttggagtctgctaatattactgtatatgggattttggtgggaccatccctaaggatttaataataaaatgtccctttatattgttgagaattttaaataattctttaaagcagttatgttctgataaatatttaataactggctcttgagtggcatggggcgctgatttgcagtgtttgccaattcctgtggtgtaaatactcccactgtggctgatttcaaggtacagatgtgataccactgaatgtgaagctgagaagagatgcatgcaattggctctgactcatgcggttgatacatgccagctccagcacatcatgacttcaagctgtcccagatgtgccctgtctgaatttctgacctagatgactggttgttggcaggaagtctcagctcctcattccatggccttctccacagaattgcttgagtgtcttcacggcatggttgccagtcaccccgtgctaggtatgggtagagggctctgcacttgtccaggttccagccaacttcatgaaggatttttattgcctgactccgagtaaaaggttagctaaatctgggctgcaaggtgcaaagtccttgagagcatctgcttgagcaaagtatgtgagcgccccaatctttatgggtacccagatgtccatcatctgtgctgcaatatggctgagtgggaggtagctgaccaccatctcatgcttgtctgtcagttgaaagtcctttgccactgctcctgccatccacgtgatctacatcgagtaccaccagcagtgtctcggcgtcgagaagtctttcttcaaagtaccgccaggcggtccgcgcctgcgcgcccctccc

SEQ ID NO: 10882 - RNA, 2129 nt, Homo sapiens
  source 1..2129: mol_type = other RNA
ctgaatagctgggactacaggtacgtgtcaccacatcgcgttaattttcaaatttttaggagagatgaggtctcactatgttgctcaggctggcctcaaactcttgacctcaagcgatccccccgtgttggccttccaaaatgctggaattacaggtgtgagccaccatgcctggcctaattttgcttacacacacacacacacacacacaagaaaattgcaatttcaggagccatgacttatgacatcattgattcctgatggggcagctcaaaaaaaacaaaacaaaacaggaccataagatggcagtattgcataacaagctttactgcacggcacttagataggtttgcatgcggggaatgtcccttccagcaggactccttccagaggaactcctgggacagaggagagttagaggcagggcttaagtgtctaggtgatgtcattgagtagcaaggtggggagagtctgcatcatagaactctgaaaggcaacaataatttggggtttcttatggctgtaagatttttcttctctgtgattaataggtgttgttgggtgcaattttatggggtatgcaaagcaggtgggctctaaatgactaaacatatgcttatttgtgcaatatttatagcaatggattgtgtgagaatttgagcttggtgctggtgggctttgagctgagaggtccctgcctgcctgctgtaaagaaataaatgagatagggctgatagaaagacactgtctttggctcacttatacagcaagtgacaaccaatttagttcagacctttcttgcttctagacctgcaccatccactcttatccacttctcattcttcctggaagctgccacggaacatgcagacccccgtatccacttttgccagtagggacacccacttttgaaaagccacggacccctggcaacgcagctgcagacataccatttaactcaccctgcctggaaaaggaaagtaaatgttttcttcccaatttttgctagggaaatccaggcacatatatgtattcagtaactcaatgatataaatttcagggcttgtgtctgtgtgttattggaaaagcatttgaggctggctgtcatggttcatggctgcaatctcaacactttggaggctgaggcaggaggctcacttgaggccaggagttccagaccaggctggacaactctacctctacaaaaaaataaaataataagccccgcatggtggtgcacacctgtagttctagctactcaggaggctgaggtgggaggattgcttgagcccaggaattcaaggctacactgagctatgatcacaccactgggcctgggcaatggagtgagattctgtctctaaaaaaaaaatgcatttgagaattttagcaaatctaagtacatttggagtctgctaatattactgtatatgggattttggtgggaccatccctaaggatttaataataaaatgtccctttatattgttgagaattttaaataattctttaaagcagttatgttctgataaatatttaataactggctcttgagtggcatggggcgctgatttgcagtgtttgccaattcctgtggtgtaaatactcccactgtggctgatttcaaggtacagatgtgataccactgaatgtgaagctgagaagagatgcatgcaattggctctgactcatgcggttgatacatgccagctccagcacatcatgacttcaagctgtcccagatgtgccctgtctgaatttctgacctagatgactggttgttggcaggaagtctcagctcctcattccatggccttctccacagaattgcttgagtgtcttcacggcatggttgccagtcaccccttgagagcatctgcttgagcaaagtatgtgagcgccccaatctttatgggtacccagatgtccatcatctgtgctgcaatatggctgagtgggaggtagctgaccaccatctcatgcttgtctgtcagttgaaagtcctttgccactgctcctgccatccacgtgatctacatcgagtaccaccagcagtgtctcggcgtcgagaagtctttcttcaaagtaccgccaggcggtccgcgcctgcgcgcccctcccgcccctcc

SEQ ID NO: 10883 - RNA, 601 nt, Homo sapiens
  source 1..601: mol_type = other RNA
ctgaatagctgggactacaggtactcgccaccacacctggcatatagggaagtgtggtcacagaacaccaggcatctgcctaaatccagtgtcactcagaaggctgaggtcactcctgtccagggccagaatctgtcctaacttcaaaggttctgcatgggtcaagcactagagtcactggcacacttggtgctgcacatacagtcagtgtcacacaaacataaccacacatccactcttttatttttttgagacagggtctcgctctgtcacctagactggaatgcagtggttcaaacacggctcactgcagccttgacctctcaagctcgagatcctcccacctcagcttcccgggtagctgggaccacaggtgtgggccaccacactcagataatttttaattttttgtttgtttgtttttgagacgaagtctcgctcttgtcccccaggctggagtgcgatggcgcgatctcggctcactgcaacctctgcctcctgggttcaagcgattctcctgcctcagccccctgagcagctgggattacaggcacctgccaccacgcccagctaatttttgtatttttagtagagacagggt

SEQ ID NO: 10884 - RNA, 2409 nt, Homo sapiens
  source 1..2409: mol_type = other RNA
ctgaatagctgggactacaggtatataccactgcacccagctgtaagaccaagccacctttaatgaacaaatatccttcctgttctgctaaagtacagaaactatttctactaggagccagtgggaacctaggggttatctggagcttagctccagctaagtgacaggaaagggagggtctagaccagtccctgctgatgtgctgctccacattgtcaaagcccaaggagagatgaggcctctgggaccagagagggccctggtgctaaggtggtggtggaacagaacccagcagccttcagctggatactgatagcttcatctcctgaaggctttcagatgacagcagctggacccaccgttttacctacctgtgtccactcacatgggctcaggatgtggacttagaggctctcctttaataaatatcttatacaatgattctgtctttggctctgtttttcctgtgcaggcccgcagagtgccaggtgcctctctcccctcctctactattttggctcctgctatgaaaagaatagtaaaactactttatagagaggagacgctttagctggagaacaactctgtcttcctaggaaccagggacagtcaataaccagaaaggacagagggctaaagggccttggctaatcttactatcagatgggtggcagacaagttaccagagagaagcagactatcactttttcacatggtcaaagcagataggcacagaaaagcatctatgatcccctgaaagtccttggagatggcactggatatccccaaattttcttatcagagggtagaaaacttgaaaagagtctttttttgagacaaagttttgctcttttgcccaggctggagtgcagttgcacgatcttggctcactgcaacctctgccttccggtttcaagtgattctgctgcctcagcctcccgagtagctgggattacaggcgcatgccaccacacccagctaatttttgtatttttagtagagacaaggtttcaccatgttgaccaggctggtcacgaactcctgccctcaagtgatccacccacttcggcctcccaaagtactgggattacaggtgtaagccactgcgcccagccggcaggtccatgttttaaaagccagataaaactacagctctctccacattcagacgggacagccagccctgatggagctggggtgaaatgcccccttcagactgaccaggtgctcagtacagaaaggccaggtgccactccagggaatctaaggtgcctcaagaaaatgccaggtcagattttcctcaagaaagaccagccaggcacaggctcacatctgtaatccaagtgctttgggaggccaagaagggaggatcgcttgagcccaggagttcaaaaccaacctggaccaacagtgagactctgtctctaccaaaaaaaaaacaaaaaactaaccaagggcagaatctgatggcagcccctgaaagaatctgggggaaactggaggatatgagtgtgtgtgtatgaagttaacttcaaagcaagcttcctgtgctgagggggtgggaggtaagggtgtgatgaggcagggcttctcctttggcaaagcctctgtagtccttccttagtcaccagggagttgtgggagatatagaccagggttgcaggtgcctggagtacagggacagcagacaggtcatggtgggtgaggggtcagctggtggggcacagatgcgtttcctcggcagtccacatattcatagctctgaaagaccagctgctctgaatggctcaggtatgaacaggtcagggtgccctggatgtgcaaaagcacatggtggactttgatttccagccaggtacagattttgtatgtgttttcatcccgtatcttggtagctactgcgtaaaacatcgttatgttgaggtagatatcagcctcatcaaaggccactgtggaggagttgaggcctgcaggctgcacaatgacggaccggggaaacaggaaaaagacgatgaaggaggaggtcaccaggcagatgagcacggccaggaacacaaagagcttcgtgtgcttgggcttcagcctctggtccccatagggaatgagagccaccaactgcttctccagctcttggggaatcttgccactgccctggcaggtgggacaagtcacgaagctggcatcagcagttccttcacaaggcacacaggaacaaaaagacttgctgctaccggtgctggagtagttgacagccttgctgccaatggctggtttggaggacaggattgacttgttctcatcctcccgccaagagcccagctgggaaaacgtcttacccattcttcaggggcgggggtttcaccgcggacgactgcagcgacagaaacggaagagagtggaatcgaaaat

SEQ ID NO: 10885 - RNA, 2574 nt, Homo sapiens
  source 1..2574: mol_type = other RNA
ctgaatagctgggactacaggtatataccactgcacccagctgtaagaccaagccacctttaatgaacaaatatccttcctgttctgctaaagtacagaaactatttctactaggagccagtgggaacctaggggttatctggagcttagctccagctaagtgacaggaaagggagggtctagaccagtccctgctgatgtgctgctccacattgtcaaagcccaaggagagatgaggcctctgggaccagagagggccctggtgctaaggtggtggtggaacagaacccagcagccttcagctggatactgatagcttcatctcctgaaggctttcagatgacagcagctggacccaccgttttacctacctgtgtccactcacatgggctcaggatgtggacttagaggctctcctttaataaatatcttatacaatgattctgtctttggctctgtttttcctgtgcaggcccgcagagtgccaggtgcctctctcccctcctctactattttggctcctgctatgaaaagaatagtaaaactactttatagagaggagacgctttagctggagaacaactctgtcttcctaggaaccagggacagtcaataaccagaaaggacagagggctaaagggccttggctaatcttactatcagatgggtggcagacaagttaccagagagaagcagactatcactttttcacatggtcaaagcagataggcacagaaaagcatctatgatcccctgaaagtccttggagatggcactggatatccccaaattttcttatcagagggtagaaaacttgaaaagagtctttttttgagacaaagttttgctcttttgcccaggctggagtgcagttgcacgatcttggctcactgcaacctctgccttccggtttcaagtgattctgctgcctcagcctcccgagtagctgggattacaggcgcatgccaccacacccagctaatttttgtatttttagtagagacaaggtttcaccatgttgaccaggctggtcacgaactcctgccctcaagtgatccacccacttcggcctcccaaagtactgggattacaggtgtaagccactgcgcccagccggcaggtccatgttttaaaagccagataaaactacagctctctccacattcagacgggacagccagccctgatggagctggggtgaaatgcccccttcagactgaccaggtgctcagtacagaaaggccaggtgccactccagggaatctaaggtgcctcaagaaaatgccaggtcagattttcctcaagaaagaccagccaggcacaggctcacatctgtaatccaagtgctttgggaggccaagaagggaggatcgcttgagcccaggagttcaaaaccaacctggaccaacagtgagactctgtctctaccaaaaaaaaaacaaaaaactaaccaagggcagaatctgatggcagcccctgaaagaatctgggggaaactggaggatatgagtgtgtgtgtatgaagttaacttcaaagcaagcttcctgtgctgagggggtgggaggtaagggtgtgatgaggcagggcttctcctttggcaaagcctctgtagtccttccttagtcaccagggagttgtgggagatatagaccagggttgcaggtgcctggagtacagggacagcagacaggtcatggtgggtgaggggtcagctggtggggcacagatgcgtttcctcggcagtccacatattcatagctctgaaagaccagctgctctgaatggctcaggtatgaacaggtcagggtgccctggatgtgcaaaagcacatggtggactttgatttccagccaggtacagattttgtatgtgttttcatcccgtatcttggtagctactgcgtaaaacatctgttcactggccaaagggccaatgtgtaggagaaggttgttggaaacctgccccaccacgagggacaggtgcagaacctcgagggtcagctgtgtcaccataatggggtagtagttgccattggagatgtttaagatattcgttatgttgaggtagatatcagcctcatcaaaggccactgtggaggagttgaggcctgcaggctgcacaatgacggaccggggaaacaggaaaaagacgatgaaggaggaggtcaccaggcagatgagcacggccaggaacacaaagagcttcgtgtgcttgggcttcagcctctggtccccatagggaatgagagccaccaactgcttctccagctcttggggaatcttgccactgccctggcaggtgggacaagtcacgaagctggcatcagcagttcccattcttcaggggcgggggtttcacttgttcaggtctgggatcccaggctcctcagccgcacgagggcgagacttctggagtgcgtctttggggagaagggcctctaagggcagagtgggctgggctgggctgagctgagctgggcggtggtggggagaagcaccgcctggggccggcaaccggccggagtcccgcggacgactgcagcgacagaaacggaagagagtggaatcgaaaat

SEQ ID NO: 10886 - RNA, 2718 nt, Homo sapiens
  source 1..2718: mol_type = other RNA
ctgaatagctgggactacaggtatataccactgcacccagctgtaagaccaagccacctttaatgaacaaatatccttcctgttctgctaaagtacagaaactatttctactaggagccagtgggaacctaggggttatctggagcttagctccagctaagtgacaggaaagggagggtctagaccagtccctgctgatgtgctgctccacattgtcaaagcccaaggagagatgaggcctctgggaccagagagggccctggtgctaaggtggtggtggaacagaacccagcagccttcagctggatactgatagcttcatctcctgaaggctttcagatgacagcagctggacccaccgttttacctacctgtgtccactcacatgggctcaggatgtggacttagaggctctcctttaataaatatcttatacaatgattctgtctttggctctgtttttcctgtgcaggcccgcagagtgccaggtgcctctctcccctcctctactattttggctcctgctatgaaaagaatagtaaaactactttatagagaggagacgctttagctggagaacaactctgtcttcctaggaaccagggacagtcaataaccagaaaggacagagggctaaagggccttggctaatcttactatcagatgggtggcagacaagttaccagagagaagcagactatcactttttcacatggtcaaagcagataggcacagaaaagcatctatgatcccctgaaagtccttggagatggcactggatatccccaaattttcttatcagagggtagaaaacttgaaaagagtctttttttgagacaaagttttgctcttttgcccaggctggagtgcagttgcacgatcttggctcactgcaacctctgccttccggtttcaagtgattctgctgcctcagcctcccgagtagctgggattacaggcgcatgccaccacacccagctaatttttgtatttttagtagagacaaggtttcaccatgttgaccaggctggtcacgaactcctgccctcaagtgatccacccacttcggcctcccaaagtactgggattacaggtgtaagccactgcgcccagccggcaggtccatgttttaaaagccagataaaactacagctctctccacattcagacgggacagccagccctgatggagctggggtgaaatgcccccttcagactgaccaggtgctcagtacagaaaggccaggtgccactccagggaatctaaggtgcctcaagaaaatgccaggtcagattttcctcaagaaagaccagccaggcacaggctcacatctgtaatccaagtgctttgggaggccaagaagggaggatcgcttgagcccaggagttcaaaaccaacctggaccaacagtgagactctgtctctaccaaaaaaaaaacaaaaaactaaccaagggcagaatctgatggcagcccctgaaagaatctgggggaaactggaggatatgagtgtgtgtgtatgaagttaacttcaaagcaagcttcctgtgctgagggggtgggaggtaagggtgtgatgaggcagggcttctcctttggcaaagcctctgtagtccttccttagtcaccagggagttgtgggagatatagaccagggttgcaggtgcctggagtacagggacagcagacaggtcatggtgggtgaggggtcagctggtggggcacagatgcgtttcctcggcagtccacatattcatagctctgaaagaccagctgctctgaatggctcaggtatgaacaggtcagggtgccctggatgtgcaaaagcacatggtggactttgatttccagccaggtacagattttgtatgtgttttcatcccgtatcttggtagctactgcgtaaaacatctgttcactggccaaagggccaatgtgtaggagaaggttgttggaaacctgccccaccacgagggacaggtgcagaacctcgagggtcagctgtgtcaccataatggggtagtagttgccattggagatgtttaagatattcgttatgttgaggtagatatcagcctcatcaaaggccactgtggaggagttgaggcctgcaggctgcacaatgacggaccggggaaacaggaaaaagacgatgaaggaggaggtcaccaggcagatgagcacggccaggaacacaaagagcttcgtgtgcttgggcttcagcctctggtccccatagggaatgagagccaccaactgcttctccagctcttggggaatcttgccactgccctggcaggtgggacaagtcacgaagctggcatcagcagttccttcacaaggcacacaggaacaaaaagacttgctgctaccggtgctggagtagttgacagccttgctgccaatggctggtttggaggacaggattgacttgttctcatcctcccgccaagagcccagctgggaaaacgtcttacccattcttcaggggcgggggtttcacttgttcaggtctgggatcccaggctcctcagccgcacgagggcgagacttctggagtgcgtctttggggagaagggcctctaagggcagagtgggctgggctgggctgagctgagctgggcggtggtggggagaagcaccgcctggggccggcaaccggccggagtcccgcggacgactgcagcgacagaaacggaagagagtggaatcgaaaat

SEQ ID NO: 10887 - RNA, 2740 nt, Homo sapiens
  source 1..2740: mol_type = other RNA
ctgaatagctgggactacaggtatataccactgcacccagctgtaagaccaagccacctttaatgaacaaatatccttcctgttctgctaaagtacagaaactatttctactaggagccagtgggaacctaggggttatctggagcttagctccagctaagtgacaggaaagggagggtctagaccagtccctgctgatgtgctgctccacattgtcaaagcccaaggagagatgaggcctctgggaccagagagggccctggtgctaaggtggtggtggaacagaacccagcagccttcagctggatactgatagcttcatctcctgaaggctttcagatgacagcagctggacccaccgttttacctacctgtgtccactcacatgggctcaggatgtggacttagaggctctcctttaataaatatcttatacaatgattctgtctttggctctgtttttcctgtgcaggcccgcagagtgccaggtgcctctctcccctcctctactattttggctcctgctatgaaaagaatagtaaaactactttatagagaggagacgctttagctggagaacaactctgtcttcctaggaaccagggacagtcaataaccagaaaggacagagggctaaagggccttggctaatcttactatcagatgggtggcagacaagttaccagagagaagcagactatcactttttcacatggtcaaagcagataggcacagaaaagcatctatgatcccctgaaagtccttggagatggcactggatatccccaaattttcttatcagagggtagaaaacttgaaaagagtctttttttgagacaaagttttgctcttttgcccaggctggagtgcagttgcacgatcttggctcactgcaacctctgccttccggtttcaagtgattctgctgcctcagcctcccgagtagctgggattacaggcgcatgccaccacacccagctaatttttgtatttttagtagagacaaggtttcaccatgttgaccaggctggtcacgaactcctgccctcaagtgatccacccacttcggcctcccaaagtactgggattacaggtgtaagccactgcgcccagccggcaggtccatgttttaaaagccagataaaactacagctctctccacattcagacgggacagccagccctgatggagctggggtgaaatgcccccttcagactgaccaggtgctcagtacagaaaggccaggtgccactccagggaatctaaggtgcctcaagaaaatgccaggtcagattttcctcaagaaagaccagccaggcacaggctcacatctgtaatccaagtgctttgggaggccaagaagggaggatcgcttgagcccaggagttcaaaaccaacctggaccaacagtgagactctgtctctaccaaaaaaaaaacaaaaaactaaccaagggcagaatctgatggcagcccctgaaagaatctgggggaaactggaggatatgagtgtgtgtgtatgaagttaacttcaaagcaagcttcctgtgctgagggggtgggaggtaagggtgtgatgaggcagggcttctcctttggcaaagcctctgtagtccttccttagtcaccagggagttgtgggagatatagaccagggttgcaggtgcctggagtacagggacagcagacaggtcatggtgggtgaggggtcagctggtggggcacagatgcgtttcctcggcagtccacatattcatagctctgaaagaccagctgctctgaatggctcaggtatgaacaggtcagggtgccctggatgtgcaaaagcacatggtggactttgatttccagccaggtacagattttgtatgtgttttcatcccgtatcttggtagctactgcgtaaaacatctgttcactggccaaagggccaatgtgtaggagaaggttgttggaaacctgccccaccacgagggacaggtgcagaacctcgagggtcagctgtgtcaccataatggggtagtagttgccattggagatgtttaagatattcgttatgttgaggtagatatcagcctcatcaaaggccactgtggaggagttgaggcctgcaggctgcacaatgacggaccggggaaacaggaaaaagacgatgaaggaggaggtcaccaggcagatgagcacggccaggaacacaaagagcttcgtgtgcttgggcttcagcctctggtccccatagggaatgagagccaccaactgcttctccagctcttggggaatcttgccactgccctggcaggtgggacaagtcacgaagctggcatcagcagttccttcacaaggcacacaggaacaaaaagacttgctgctaccggtgctggagtagttgacagccttgctgccaatggctggtttggaggacaggattgacttgttctcatcctcccgccaagagcccagctgggaaaacgtcttacccattcttcaggggcgggggtttcacttgttcaggtctgggatcccaggctcctcagccgcacgagggcgagacttctggagtgcgtctttggggagaagggcctctaagggcagagtgggctgggctgggctgagctgagctgggcggtggtggggagaagcaccgcctggggccggcaaccggccggagtcctaggggaacgaatgtgccgcaccgcggacgactgcagcgacagaaacggaagagagtggaatcgaaaat

SEQ ID NO: 10888 - RNA, 1205 nt, Homo sapiens
  source 1..1205: mol_type = other RNA
ctgaatagctgggactacaggtatgagccaccacaccggaccgtcctaaagattaatgatcaatctacggcctaagcaatccaagccataagcagtgtctgaagattaggtaaagatgcaatgtgcctgcagatgagccctaagtccatttctgctacttcaaaagttattgcagggagcttcagttctagcgagtgctttccacacaaacctgcaaatatgtcttttttcttaactttaggtctatggagaaaaggttgaaaggcccaaaatgactgatgaacatgatatataatgacagctggctcttaaagattctgttagcccctggtattaggaaatccaagtgaaaggccctgattatgctaagggttgcaaagatgcccaataatatttgaatttcaaatgaacaacaaataagtttaacataactatgtcataaatattgcacggaacacactttcactagaaaaatatatctttagctgaaattcaaatttaactgggtatcttgtatttttatttgctaattctggtaactaatatagcttacatgaactcttgcaaaatatccaaaatgcatttctgcttctcgcttaaggaaagacttctggttgtcctggaatttgaggtgcttgaaggtctgctgtcagctcaactttgcatcttctttctctgggatgcccctcccataccatttttagtcacgcaaaatctcttgtacttttgagcaggtcatatgtttctatgtttccccatcttctcgaagactgtcttcatcacctgcgtggccattgctcacttttctctttgtagaaactgtcttcaaaatctaggtcaaatatcatacatccatgattccttggctggctctccgaaaggtcaaatagtaattttttaaaaattaatgatgtctgtcttcttgttgtgaaaagaggaagcaaaacaagcaagtctctgtaagataattcattggttcttttggtctcaggccgccattttgtaacttgctcttgtacactgccttcatgacttgaaagaattaatgcatcttcaaaattctgctctgtacctaacaacagagtttgaaattccatatccagtaaaattatccttcagaaatgaagaaataaagatgttttcagataaaagttgagagaatttgtcaccaggaggcctgcctttcatgatatgttaaaatacct

SEQ ID NO: 10889 - RNA, 4586 nt, Homo sapiens
  source 1..4586: mol_type = other RNA
ctgaatagctgggactacaggtatgagccaccatgcccttctctaaagcaaacttttgactttcaaggcacagttagcagtgttgggagaatccctgaaatatgttaatgttttaacattggcttattttagaatgagagggctcagaatagcttatgaaatcaaacagtggtgatcaaagagaagcttaagttgtctccccactccatttcattttatgaatgatttactaaaaatgccactttttctcagtttgcatgtgttaacttcagaatactcagagaggaaaatggcttacaatcaaatctagtactacctgaaaatgtgtctttccttaatgccacttaattagtattaatgaactttttaattttaatgtctttttattttatatttgctctacaaactacaaaatggtttacaataaatgttgtgtacacttaatggcacaaaatagtttagagtgttctgtaacacttattaactacagcaggccttatgtatttatgtatttatgtatttatttttatgtttttgagacagcgtctcactctgttgcccaggctggagtgcagtggcacaatctcagctcactgcaacctccacctcccaggttcaagcgattctccagcctcagcctcttgagtacctgggattacaggtgcgtgccaccacgactgactaatttttgtatttttagtagagatagggttttgccatgttagccagggtgatctcgaactcctgacctcaggtgatctgcctccctccgtctcccagagtgctgagattacagccatgagccacggtgcccagccgtcatactttatttttttcctcacccaccctccatttccgttttttcaaatagattttctctgggactgcaaggatagacatctggatataaaagagggagatttgagacttgcctatggctccaaacaatcaagaaatcaaatctggctgggcgtggtggcttatgcctgtaatcccagtgctttgggtttccgaggctggtggatcacctgaggtcagaagttcatgaccagcctggccaacatggtgaaaccccgtctctactaaaaataccaaaaaattagctgggcatggtggcgcatgcctgtaatcctagctactcaggaggctgaggcaggagaatcgcttgaacccaggaggcagaggttgcagtgagccgagatcgtgccattgcactccagtctgggcaacaagagaaaaactccgtctcaaaaaaaaaaaaaaaaaaaaaaaaaacaactacatctaatttaattttggagaacattcctaaactgaatctctttatccttatgtctgcccttattcacatttgcaaataagtgaaatccttttctttctccacccttcctcccaccatgattatttgtgaagatcaccatttaccaggcatttccatgattatgattatgaatgattgcaggcaaggtattgatcaaagataatcactcatcagggacaagaatttagagattcctgaataataaactatatctctgcttgtcaaacctaatcacttcccaatatatcaaaaagggaaggtagttctcttccctatgcatgcataactttctactggaaaataatttagaggcaaataaaaggatctctctatggaactaagtatttcctgggccaggaccaatgaacttctaaggaaaatgtgaataatggcttattcattacttgctagcacagagatggaaaagcagaagttcctaccacatatgcatttatagagggtgacatttctttaaacagaattccaactggagaaagggttatagatatatgatctggggatcaggataactgctttgtattgagtaagcctagcctcactctaggtttcccattttcaccaaactaagtactcttatctttactaaagctgcaatctactaccagtttttgttttaatgaggatgtaacatctttgcataccaagtataaaattttgcttctcttctctcactgagcctgtaaataggagctacatatagtcatcagatacctggtcatggccctctaatctctgagacttattcctatcagaatttgggggcaaactggagccagcctccatttttatctccccagtggcatgagggaaagggaagttgggcataaaacgcttaagaaagcgaaactcactattaccagtgccagtggctgaacacatttcatatggacaaggccgagataaggatccattgccttgtccttgtaccaggttgttagagaaattacagtcatcatagaaatgctcttgaattgtgaacttttctctatatttaatcttttggtagacatgtataatgaagatcactatgacagagaggagaaagagaaaggaaaggatgaccagagaaatgaccaaatatttagtggatggatttacctttctagaatgcttggttggatcctggaactgcaggtagggctctgaaaagccatctaccagcaggatgttgagtgagacagtagtggaaagagctggttggccgtgatcctgaacaagaatgatcaatttctgcatcatggggtctctctcagatatctgccttaatgtatggatttctccattttgtctttgaacagaaaataacccaaggtcagtggccttaagtagatgatatgaaagccaagaattctgacctgagtcaccatccacagccaccactttggtcactaggtagcctgcctctgcagacctgggcaccaggtcattgcagggcaaggtgccgttctgcagtgggtataagatcattggacgattgtcattgtcatctaggacaaccactctgacagtaacttggctactcagtgacaggaagcccccatcagttgcctttaccacaaattgaaaatcttgaatggcctcataatccatggttctcagcgcgtagagcttcccattgcctgaatttatggatatgtaagcaaagactgaaagatctccgttttttggaggcaacagagaatatgttatttgggcattctcacccaaatcaagatcctcagcatggactttgccaataaaaaccgcaggactgttgttttctcgaacagtcaagatataggaatcttcccgaaatattggaggattgtcattaacgtcggatattagcacctctatcatagtctcggcagacaagctaggtggtccagtatccatggcaacaatggtgatattatagcctgagacctcctcccgatccaagcttctgtcagtgaccagtgagtaagaattcccaaatgtaggtttgattacaaagggaaggtcttctctgaggaagcaggtgacttttcctcccactcgaatgtcccggtctctgatagtgaaaagggctactactgtctgtggtggtgagtcttcagggagtgggctggacacagaggagaccatcacttcgggaggattgtcattcacatccaccacttctaccaggactttgctgtgggcagagaggcctccaccatctgtagcttgaatgtcaatgtcgtatgtttcaatggcttcaaaatcgaggggtcctcttagtcgaacttctccattttgagggtcaatctgaaacgtcttgagaattgcttctgggttttgagctaaagagtaagttatcgctttgttggtgccctcgtctaggtccacggcagtcaccgtggccaccaaagagccattggggctgttctctgatacctgggctctgtacaccagtcgcgagaactggggcacgtggtcgttgacatccagaaccaccacgtggatgtgagctgtgccagacttaggcggggacccgccgtccaccgccgtaattgtcaagttgacttcaggctgctcctctcggtccaggggtttgttcagcaccagctcagcatatttaggcccgtggctgcagaagcgggtgtgcaggtggaaatacccattggcactcagggtgtagttctggagaccgttaaggcccacgtccagatcctgggcgctctgcagaggaaaacgtgaacccaaaggggtgctctccggaatctttaaaagcggctccttgtttaggaaaactggggcattgtcattgatatcaaataccctgacctcggcccggaaggactgcagcggctccaccaggactacttcaaagtgcagaacacaagggtcggctttgccacaaagtgactcccgatccagtttctccttcacaaacaaatctcccgtcttgcggtggagccggaaatgcattttgttgccctcggaaaccagccgcgccccgcgcgcagccagcttccctacctccagtcctaggtccttagctacgttggccacaaacgagccgctctccatttcctctgccactgaatagcggatagttgtcgcatcccccacagatatgcacagaaaaatgagaagagatcccacttgcctgttttgcaaagattttctgcgcgtacccgccatcagttctcacaagcgcgctctctgcaatcagagccaactgttgcggatatactttcacttttctgcaacaggttactgcaacagctgctctccgctt

SEQ ID NO: 10890 - RNA, 2279 nt, Homo sapiens
  source 1..2279: mol_type = other RNA
ctgaatagctgggactacaggtatgcacaatgacacccgactaatttttataatttgtgtaaattccatacagacagggtttcactatgttgcccaagctggtctcaaactcctggccttaagcaatcctcccaacccaggttcccagagtgctgggactacaggaacaagccactgcacctagcctagatgaaattttttaatgtgacacaggttttctgaatacaatgcattgctccaacaacttcaaagtcattgtggattcctgcaataaattcgctcccacatcttctccatgtttcttcttttaaagtctcaagttactaggtaggaagaactaaagatactgaatgtagacacccccggcccccggatatcttattcccccaaactatacaatgcatatgagatgatttttttaaaaatgcatgcaacatacccttcagatgttgtccccaagagaagggaagataatttgagaaactgaattgaaaaataaaaataataggctctgtgaagtatgtatatttacatcactgcacaatttgtgcatctgccataatgacttctatatatacacacacacacacacacacaatttgtggttataatcaaataagtccagttcaaacttataaagtctatgagaaaaaccaagacaacaccaaaagataagataaaatctataacgaaacaattttcaaaaccttcctacagtgtggaattctggttgcttaaataatgccagttccatgaatttcaactgtgctctgatctatttctatacacacaggtacagagaaaactggaaatgtcctcaggccgtgaagaagacattttgcttctggtctgcttaggtgcagttctttgttccaggcagattccaatcttcctgtttcttccagatgtgagctcgtcctcagaaattcttgaagatttctaaatccttctgcggcacgggcgcggctgtgtcccagtcatgctcagggtaagtttcgaagttggaagtgtcgccgttgccagctatcgtgggcacgatgggaggcttcagttttctctgcggaacagctttccagtccacggagcggaaccaccgatggtgtttcacatcattcgccccgtttttacatggaaatccaaatgtctggggaaatatagtttgcctgcaagaattttctgataaatgccaaacgggttgtcatcaaaaaatggaggaaaccccgaaagcatctcgaatatcaggatgccgagggcccaccagtccacggcccttccgtggcccttgctctgaatgacttcgggggctaggtactcgggtgttccacagagggtccaagtcctgtctaccagcttcttggcaaacccaaagtccgtgagcttgatgtgaccatccctatccagcaggatgttctccggcttcaaatccctgtagacgatctccttggagtgcaggtactcaatggcacagatgatctccgcagagtagaagagccccgtggtgctggagaagtgcccccggttgcgcaggtagctgaagagctcgccacccggcacatactccatgagcatgtagaggaagcgctcctcatgccacgtccagaacagcctgatgaggaacgggtggctgacttccttcaggacagacttctcattgtgcacgtgctgctcctgcttccggcggatgacgtcgggaatgctcatcaccttgagggcgaagaaatgcttggctgtcttctccttcaccaggtgcacccgcccgaacgtcccagtgcccatggtgaccagcgcgtcgcagtcctgcaggcggtaggcaggcgcctccggcgaccgcgcctcggggctggggcagagcgcgggcgcccagtcggcggcatcctccgtcacctctcgggagttgctctccgccgcggccgcctgggccggcccgggcgcctccatggggaggcactcaggtccggggcgccgggccaggccggagcgctcgggaagccggactccccgggacgcagcctcggagggcggcgcggcagccgcggcagcatcaacggaggctccccatgcgcgccctcgcctctgggtgcgcggctcggcacggctgacggagacacagagacaatggctgggcggtgctcacggcactagcagcaatagccccgggagggagcagccgctggcctcgcggggcgtgcaccgagtgctggatggctgcgaggaaggcgggggccccaagcattcccggtctcacgcccgccgcctcctccagctcggtggccgcgtgc

SEQ ID NO: 10891 - RNA, 2838 nt, Homo sapiens
  source 1..2838: mol_type = other RNA
ctgaatagctgggactacaggtatgcaccaccacacccagctaatttttaaattatttgtagagacaggggtttccctaggttgcccaggctggtcttgaactcctgggctcaaacaatcctcctgcctcagcctccaaagggctgagattacaggcacaggccactatgtccagcttgagtttgattttttttaaagagaaaatcaacaatcccttaatgagcctgattttaagacttaatgtgtcaaaatatgcagttcttaagacaaagggggaataggtgtaaaagaggtccttggtgttcacagcctaaacctggactcagggttggctgctatcagggttgaggggtccctaccgctggacaccttagatggcctgagaaccaagcccacatcagtgctatggtctagccattctccctcaaagggacccagcctccctccagccagcctgaggcccactggcatgcagggacctctgagaacgactgactcccagggattccttggctccttaccttccagcattctcctgcaaccaagcccagggcacatgggactgtccctgagccaaggacccaggcatgctgtgagccaggggaaggggagtaaagagactggtggcttttaccctccatctgagggtggaggggctgggaagggacaggaggtctgtgggaggtcactccagaggctgggaagggacaggagggattctgttgttctcaagtgacctatttgacttccccctcctgaggagtcagcacacaggctgaaagatgcagtgagacacaagtttattggtggagctgcagcggagtcctccctctttcagggatagccaagggcacagcaccaacagagggatggagagatagacccccaaacagacacatggatggagcagactcatagaaaccatagcacagccacataggcacagagacacacaggccacagcaccaagaacacacacacacacacacacacacacacacacacacacacagacaaaaccacagggctaagacacacggacaaagtgcgggctttggggcccctgcatagacagagcgagggccatgtggggagggggcccctactgacctcccccaggcataggcacaccaacagcacatagacaggcagatgcccccagccagccagcctgccacacagacaaatggactgcagggaaaggatgttcgtggctccacatgaaccatggggagatggcaccacaggccttcaacacaccctgccacactgaggcctgggagtccccgcccctgaactagtcacatctattcccctgactcccaccccactccccgccacactttggtcttgcccactggggctggggctggggctgaggctggggaaactggcaggtggtaggagggagagaggaaggggtatggacctggctcggtcccgtctctgtgatcagggcagcagatgctgagagtctggggctgagcctcggcctggcagtggggtgagggcagggccatggctcaggcttgggggggttcctggcagcgcaggcactgggccatctccggctgatactgctcgacctgcagggtgcagctggagaatccaaaccgggagtagagccgggatgaggcttcagccaggacggcttcagggtcagcggtggagtcgatggccaggtgtgcagaggcaacatggtaagtgagcgtaagggcccacaggtgcagctcatgggttgcccggactcctggcaccgacaacagcgtatcccgcacaggttcgaaccccacattgcggggggtaccttccatgaggattcgaagaacgtctcggagggtgggagcggtggatccaagggcacagatggagaagaggaaggtgctgatggggtcggctgccttgtattgaggcttgaagtagatgaggatggaggcagccagtaccccaaagctctgcaggaggtcccccagcacgtgcacaaatgccgcccggacgctggtgttccccaggggcaggggctcttcaggcccctcctccagcggtgcatactctgctcccctagacccgtggctgtgggggggcccagcctggtgcagcacaaaggccattaacaggttggcacagactgcgatgctggcggtcagcagcatggcacccccctcgatgtggtagtcgctgtgcagcaggcggacgaaggccaggtacaggaggatgccagtgaccatccagagggagaccacagaggccaaagcccccagagtctctgaacggtgccagccaaaggtcatggtgcgggtggctggacgggtggagagccagagggagaagaggctgcccatcatgctgcccacatccgccagcaagtgggctgcatcggtcatgatggccaggctgtgtgccagatacccgccgaccacctccccagccatgaagacaaagcaaacggcacaggcagcatatagctgcctccgtgcatgcagcctctcaggggtaaggcccggcggcggaagggggtccctgtggcagtggtggaagggcatctccacaggtttggactcctcagggaggggctctgagggctctgtgaagagaagcaaagtcggtggccgagcctcaagtcgaagcttcaaatgctcaatgttctctcccctcgcacctgccgccactctcatccgccacggtcagcaaacccattgtgtttcctggagtgagttgggccatcaagatgggtggtgccctcctgctggggaagaggggctcggtgggaatccctgccccaaggcctggcagcaacgctcctacgctgccttgggccgcaggcctgctaagccctcc

SEQ ID NO: 10892 - RNA, 2765 nt, Homo sapiens
  source 1..2765: mol_type = other RNA
ctgaatagctgggactacaggtatgcaccaccacacccagctaatttttaaattatttgtagagacaggggtttccctaggttgcccaggctggtcttgaactcctgggctcaaacaatcctcctgcctcagcctccaaagggctgagattacaggcacaggccactatgtccagcttgagtttgattttttttaaagagaaaatcaacaatcccttaatgagcctgattttaagacttaatgtgtcaaaatatgcagttcttaagacaaagggggaataggtgtaaaagaggtccttggtgttcacagcctaaacctggactcagggttggctgctatcagggttgaggggtccctaccgctggacaccttagatggcctgagaaccaagcccacatcagtgctatggtctagccattctccctcaaagggacccagcctccctccagccagcctgaggcccactggcatgcagggacctctgagaacgactgactcccagggattccttggctccttaccttccagcattctcctgcaaccaagcccagggcacatgggactgtccctgagccaaggacccaggcatgctgtgagccaggggaaggggagtaaagagactggtggcttttaccctccatctgagggtggaggggctgggaagggacaggaggtctgtgggaggtcactccagaggctgggaagggacaggagggattctgttgttctcaagtgacctatttgacttccccctcctgaggagtcagcacacaggctgaaagatgcagtgagacacaagtttattggtggagctgcagcggagtcctccctctttcagggatagccaagggcacagcaccaacagagggatggagagatagacccccaaacagacacatggatggagcagactcatagaaaccatagcacagccacataggcacagagacacacaggccacagcaccaagaacacacacacacacacacacacacacacacacacacacacagacaaaaccacagggctaagacacacggacaaagtgcgggctttggggcccctgcatagacagagcgagggccatgtggggagggggcccctactgacctcccccaggcataggcacaccaacagcacatagacaggcagatgcccccagccagccagcctgccacacagacaaatggactgcagggaaaggatgttcgtggctccacatgaaccatggggagatggcaccacaggccttcaacacaccctgccacactgaggcctgggagtccccgcccctgaactagtcacatctattcccctgactcccaccccactccccgccacactttggtcttgcccactggggctggggctggggctgaggctggggaaactggcaggtggtaggagggagagaggaaggggtatggacctggctcggtcccgtctctgtgatcagggcagcagatgctgagagtctggggctgagcctcggcctggcagtggggtgagggcagggccatggctcaggcttgggggggttcctggcagcgcaggcactgggccatctccggctgatactgctcgacctgcagggtgcagctggagaatccaaaccgggagtagagccgggatgaggcttcagccaggacggcttcagggtcagcggtggagtcgatggccaggtgtgcagaggcaacatggtaagtgagcgtaagggcccacaggtgcagctcatgggttgcccggactcctggcaccgacaacagcgtatcccgcacaggttcgaaccccacattgcggggggtaccttccatgaggattcgaagaacgtctcggagggtgggagcggtggatccaagggcacagatggagaagaggaaggtgctgatggggtcggctgccttgtattgaggcttgaagtagatgaggatggaggcagccagtaccccaaagctctgcaggaggtcccccagcacgtgcacaaatgccgcccggacgctggtgttccccaggggcaggggctcttcaggcccctcctccagcggtgcatactctgctcccctagacccgtggctgtgggggggcccagcctggtgcagcacaaaggccattaacaggttggcacagactgcgatgctggcggtcagcagcatggcacccccctcgatgtggtagtcgctgtgcagcaggcggacgaaggccaggtacaggaggatgccagtgaccatccagagggagaccacagaggccaaagcccccagagtctctgaacggtgccagccaaaggtcatggtgcgggtggctggacgggtggagagccagagggagaagaggctgcccatcatgctgcccacatccgccagcaagtgggctgcatcggtcatgatggccaggctgtgtgccagatacccgccgaccacctccccagccatgaagacaaagcaaacggcacaggcagcatatagctgcctccgtgcatgcagcctctcaggggtaaggcccggcggcggaagggggtccctgtggcagtggtggaagggcatctccacaggtttggactcctcagggaggggctctgagggctctgtgaagagactctcatccgccacggtcagcaaacccattgtgtttcctggagtgagttgggccatcaagatgggtggtgccctcctgctggggaagaggggctcggtgggaatccctgccccaaggcctggcagcaacgctcctacgctgccttgggccgcaggcctgctaagccctcc

SEQ ID NO: 10893 - RNA, 2958 nt, Homo sapiens
  source 1..2958: mol_type = other RNA
ctgaatagctgggactacaggtatgcaccaccacacccagctaatttttaaattatttgtagagacaggggtttccctaggttgcccaggctggtcttgaactcctgggctcaaacaatcctcctgcctcagcctccaaagggctgagattacaggcacaggccactatgtccagcttgagtttgattttttttaaagagaaaatcaacaatcccttaatgagcctgattttaagacttaatgtgtcaaaatatgcagttcttaagacaaagggggaataggtgtaaaagaggtccttggtgttcacagcctaaacctggactcagggttggctgctatcagggttgaggggtccctaccgctggacaccttagatggcctgagaaccaagcccacatcagtgctatggtctagccattctccctcaaagggacccagcctccctccagccagcctgaggcccactggcatgcagggacctctgagaacgactgactcccagggattccttggctccttaccttccagcattctcctgcaaccaagcccagggcacatgggactgtccctgagccaaggacccaggcatgctgtgagccaggggaaggggagtaaagagactggtggcttttaccctccatctgagggtggaggggctgggaagggacaggaggtctgtgggaggtcactccagaggctgggaagggacaggagggattctgttgttctcaagtgacctatttgacttccccctcctgaggagtcagcacacaggctgaaagatgcagtgagacacaagtttattggtggagctgcagcggagtcctccctctttcagggatagccaagggcacagcaccaacagagggatggagagatagacccccaaacagacacatggatggagcagactcatagaaaccatagcacagccacataggcacagagacacacaggccacagcaccaagaacacacacacacacacacacacacacacacacacacacacagacaaaaccacagggctaagacacacggacaaagtgcgggctttggggcccctgcatagacagagcgagggccatgtggggagggggcccctactgacctcccccaggcataggcacaccaacagcacatagacaggcagatgcccccagccagccagcctgccacacagacaaatggactgcagggaaaggatgttcgtggctccacatgaaccatggggagatggcaccacaggccttcaacacaccctgccacactgaggcctgggagtccccgcccctgaactagtcacatctattcccctgactcccaccccactccccgccacactttggtcttgcccactggggctggggctggggctgaggctggggaaactggcaggtggtaggagggagagaggaaggggtatggacctggctcggtcccgtctctgtgatcagggcagcagatgctgagagtctggggctgagcctcggcctggcagtggggtgagggcagggccatggctcaggcttgggggggttcctggcagcgcaggcactgggccatctccggctgatactgctcgacctgcagggtgcagctggagaatccaaaccgggagtagagccgggatgaggcttcagccaggacggcttcagggtcagcggtggagtcgatggccaggtgtgcagaggcaacatggtaagtgagcgtaagggcccacaggtgcagctcatgggttgcccggactcctggcaccgacaacagcgtatcccgcacaggttcgaaccccacattgcggggggtaccttccatgaggattcgaagaacgtctcggagggtgggagcggtggatccaagggcacagatggagaagaggaaggtgctgatggggtcggctgccttgtattgaggcttgaagtagatgaggatggaggcagccagtaccccaaagctctgcaggaggtcccccagcacgtgcacaaatgccgcccggacgctggtgttccccaggggcaggggctcttcaggcccctcctccagcggtgcatactctgctcccctagacccgtggctgtgggggggcccagcctggtgcagcacaaaggccattaacaggttggcacagactgcgatgctggcggtcagcagcatggcacccccctcgatgtggtagtcgctgtgcagcaggcggacgaaggccaggtacaggaggatgccagtgaccatccagagggagaccacagaggccaaagcccccagagtctctgaacggtgccagccaaaggtcatggtgcgggtggctggacgggtggagagccagagggagaagaggctgcccatcatgctgcccacatccgccagcaagtgggctgcatcggtcatgatggccaggctgtgtgccagatacccgccgaccacctccccagccatgaagacaaagcaaacggcacaggcagcatatagctgcctccgtgcatgcagcctctcaggggtaaggcccggcggcggaagggggtccctgtggcagtggtggaagggcatctccacaggtttggactcctcagggaggggctctgagggctctgtgaagagactctcatccgccacggtcagcaaacccattgtgtttcctggagtgagttgggccatcaagatgggtggtgccctcctggcttaagagaacgactcccaggtaaagggccagacccaggtgaggagtcggcacagggccagaggtgccctgcacactcagagctctccctttgagctccttgccttgctcggttctcctgggccgcaggcgtctaccctgctctctggggttccgctgccttttccttgccaggtctttcccacagcaacgccttttctcttccttctccagcctctgagtcctcttcctcctctccccactgtcccacctctgagggacagaagtggggtggtttgagagcag

SEQ ID NO: 10894 - RNA, 2831 nt, Homo sapiens
  source 1..2831: mol_type = other RNA
ctgaatagctgggactacaggtatgcaccaccacacccagctaatttttaaattatttgtagagacaggggtttccctaggttgcccaggctggtcttgaactcctgggctcaaacaatcctcctgcctcagcctccaaagggctgagattacaggcacaggccactatgtccagcttgagtttgattttttttaaagagaaaatcaacaatcccttaatgagcctgattttaagacttaatgtgtcaaaatatgcagttcttaagacaaagggggaataggtgtaaaagaggtccttggtgttcacagcctaaacctggactcagggttggctgctatcagggttgaggggtccctaccgctggacaccttagatggcctgagaaccaagcccacatcagtgctatggtctagccattctccctcaaagggacccagcctccctccagccagcctgaggcccactggcatgcagggacctctgagaacgactgactcccagggattccttggctccttaccttccagcattctcctgcaaccaagcccagggcacatgggactgtccctgagccaaggacccaggcatgctgtgagccaggggaaggggagtaaagagactggtggcttttaccctccatctgagggtggaggggctgggaagggacaggaggtctgtgggaggtcactccagaggctgggaagggacaggagggattctgttgttctcaagtgacctatttgacttccccctcctgaggagtcagcacacaggctgaaagatgcagtgagacacaagtttattggtggagctgcagcggagtcctccctctttcagggatagccaagggcacagcaccaacagagggatggagagatagacccccaaacagacacatggatggagcagactcatagaaaccatagcacagccacataggcacagagacacacaggccacagcaccaagaacacacacacacacacacacacacacacacacacacacacagacaaaaccacagggctaagacacacggacaaagtgcgggctttggggcccctgcatagacagagcgagggccatgtggggagggggcccctactgacctcccccaggcataggcacaccaacagcacatagacaggcagatgcccccagccagccagcctgccacacagacaaatggactgcagggaaaggatgttcgtggctccacatgaaccatggggagatggcaccacaggccttcaacacaccctgccacactgaggcctgggagtccccgcccctgaactagtcacatctattcccctgactcccaccccactccccgccacactttggtcttgcccactggggctggggctggggctgaggctggggaaactggcaggtggtaggagggagagaggaaggggtatggacctggctcggtcccgtctctgtgatcagggcagcagatgctgagagtctggggctgagcctcggcctggcagtggggtgagggcagggccatggctcaggcttgggggggttcctggcagcgcaggcactgggccatctccggctgatactgctcgacctgcagggtgcagctggagaatccaaaccgggagtagagccgggatgaggcttcagccaggacggcttcagggtcagcggtggagtcgatggccaggtgtgcagaggcaacatggtaagtgagcgtaagggcccacaggtgcagctcatgggttgcccggactcctggcaccgacaacagcgtatcccgcacaggttcgaaccccacattgcggggggtaccttccatgaggattcgaagaacgtctcggagggtgggagcggtggatccaagggcacagatggagaagaggaaggtgctgatggggtcggctgccttgtattgaggcttgaagtagatgaggatggaggcagccagtaccccaaagctctgcaggaggtcccccagcacgtgcacaaatgccgcccggacgctggtgttccccaggggcaggggctcttcaggcccctcctccagcggtgcatactctgctcccctagacccgtggctgtgggggggcccagcctggtgcagcacaaaggccattaacaggttggcacagactgcgatgctggcggtcagcagcatggcacccccctcgatgtggtagtcgctgtgcagcaggcggacgaaggccaggtacaggaggatgccagtgaccatccagagggagaccacagaggccaaagcccccagagtctctgaacggtgccagccaaaggtcatggtgcgggtggctggacgggtggagagccagagggagaagaggctgcccatcatgctgcccacatccgccagcaagtgggctgcatcggtcatgatggccaggctgtgtgccagatacccgccgaccacctccccagccatgaagacaaagcaaacggcacaggcagcatatagctgcctccgtgcatgcagcctctcaggggtaaggcccggcggcggaagggggtccctgtggcagtggtggaagggcatctccacaggtttggactcctcagggaggggctctgagggctctgtgaagagactcttcaaacgcaggctgcctccggcgccaccgcggtcccgggggctcaccaggcgagtggtctccaagcccccagcggctggagagggctccatgttcccggtgccccgaccgtctaggccccaccgaggaagagagaggccgggccggccccgcgccaagtccgagcagcccgccgacccccgggatccccgcagggcggcggggccaccagagtggagcgaactgcagcgact

SEQ ID NO: 10895 - RNA, 2274 nt, Homo sapiens
  source 1..2274: mol_type = other RNA
ctgaatagctgggactacaggtatgcaccaccatacccggctcatttttttgtatttttagtagagatggggtttcaccgtgttagccaggatggtctcaatctcctgacctcgtgatctgcccgtctcggcctcccaaagtgctgggattataggcgtaagccaccgcgcccggccaaggttttattttttaattagcctatggcacttactttattttctaatttttttccaatcataacagtaaatgaagaacctttgtttaaaaaaattacctgatgattccaattattgttcatgtacaactttatttaaaatggcaatctgagttgtcttcctgacatactctgtaccaaatcttagtactcagtttcatcaagtcctttgccaattcatatattcaaaagaaacatgataaaatgtaaaaggagaatggagtgcgttaaggaataatcaataatttaagattatcaataattttgatattaatattaatttcttagctgtcctactttaatgattttcattgaaactctggcacatctttaatagtctcatgacattactatttaaataaacatgattttcatccaaattattttattcttcttttttgtttttcctttggagacagggtctcgttctgtcgcccaggctgtagtgcagtggtgcgatcttggctctctggaacctccgcctcccaggttcaagcgatcctcccgcctcacccttccaattagctgggactacagatgcccaccaccagccccagctaacttttgtatttttagtagagacagggtttcaccaagctggtctcaaactcttgacctctggtgatccgcccacctcggcctcccaaagtgctgggattacaggtgtgagccactgtgcctggcctattttattcttatttataacggttttctcaatttgtagcttaaattgaaagtacttgcaaaatgagaataatttgtctctactacataaagaaataatttttctaccccaaatgaagataaagtcacttctcacaaaataaacattaatttagcagaattaagtttccccttatggcatctgatgcttgaggattaccaaggatccatgcaatagagcactacattttggaattagctgagaatgatcccaaatttcctctagtaaacataattttggccacaaatgaagacaaaagataaaagtaattaattctagaagaacacctctcgtcagaaattaatagatcttatttaggtttctaggaagcatttaactacataaaacttatagggaaaaatggccatatttgaaaactgctacaaggatcaatgtagagcacaggattgtaatgagcagagtcacagaacatactagagaggtatgtacagtcagtcccactggaacttgtagaatcacattcttatatactgatttatacttcatcttgttccattggcagatatcctcattctccaaagcacaaggggctgccacttctgagtgagcccagcatttcaaaatcgggaactctatagttttgtcaaaggaatcaaaccggaatctgatcattcttctggagccagcttggtcacaaaacatcaacaaatctgggttattgaccacaatcgaggcttctccatcttcactgtgcggccgatgatagcggcagtgcacaggcaaaaaggcttgaaaacagtcaatgcactgtgaatctcgtctggcataaatgagaacttcagactccttggacaaatagttaggggcctctatatcaaaattttctgaaaccatcactgcctctgttatgtttctctctcgtaatgaagccaactcatacggatccacataaagtcctgcaggaatgtcctgtttaattaagagacggcaggtgtgcaagtcctcaatgctttccccaaacttcactttgattaaaaggtctctgtggaaaccatctttcaaaacttcttgcctcaaaataatttcagaacacatggcccttatgccggcgtcagagcgcgcggcggtgaaggccgcggcgggcccgcgcgtgagcccggtcgccgccccgaggagcagccaggcggccgcccgaaccgccgccacccgagccgccaggacgccggaagccggacgcccgagaggggcgcgcggggccaggtgcggacgcaggaaggggcctggccgcccgcagctcctaccgcgcgctgccccagatttatcggctgggaccgagtgctgggtgcgcgcgcctagcgcccgcggttcccagct

SEQ ID NO: 10896 - RNA, 2220 nt, Homo sapiens
  source 1..2220: mol_type = other RNA
ctgaatagctgggactacaggtatgcaccaccatacccggctcatttttttgtatttttagtagagatggggtttcaccgtgttagccaggatggtctcaatctcctgacctcgtgatctgcccgtctcggcctcccaaagtgctgggattataggcgtaagccaccgcgcccggccaaggttttattttttaattagcctatggcacttactttattttctaatttttttccaatcataacagtaaatgaagaacctttgtttaaaaaaattacctgatgattccaattattgttcatgtacaactttatttaaaatggcaatctgagttgtcttcctgacatactctgtaccaaatcttagtactcagtttcatcaagtcctttgccaattcatatattcaaaagaaacatgataaaatgtaaaaggagaatggagtgcgttaaggaataatcaataatttaagattatcaataattttgatattaatattaatttcttagctgtcctactttaatgattttcattgaaactctggcacatctttaatagtctcatgacattactatttaaataaacatgattttcatccaaattattttattcttcttttttgtttttcctttggagacagggtctcgttctgtcgcccaggctgtagtgcagtggtgcgatcttggctctctggaacctccgcctcccaggttcaagcgatcctcccgcctcacccttccaattagctgggactacagatgcccaccaccagccccagctaacttttgtatttttagtagagacagggtttcaccaagctggtctcaaactcttgacctctggtgatccgcccacctcggcctcccaaagtgctgggattacaggtgtgagccactgtgcctggcctattttattcttatttataacggttttctcaatttgtagcttaaattgaaagtacttgcaaaatgagaataatttgtctctactacataaagaaataatttttctaccccaaatgaagataaagtcacttctcacaaaataaacattaatttagcagaattaagtttccccttatggcatctgatgcttgaggattaccaaggatccatgcaatagagcactacattttggaattagctgagaatgatcccaaatttcctctagtaaacataattttggccacaaatgaagacaaaagataaaagtaattaattctagaagaacacctctcgtcagaaattaatagatcttatttaggtttctaggaagcatttaactacataaaacttatagggaaaaatggccatatttgaaaactgctacaaggatcaatgtagagcacaggattgtaatgagcagagtcacagaacatactagagaggtatgtacagtcagtcccactggaacttgtagaatcacattcttatatactgatttatacttcatcttgttccattggcagatatcctcattctccaaagcacaaggggctgccacttctgagtgagcccagcatttcaaaatcgggaactcttggtcacaaaacatcaacaaatctgggttattgaccacaatcgaggcttctccatcttcactgtgcggccgatgatagcggcagtgcacaggcaaaaaggcttgaaaacagtcaatgcactgtgaatctcgtctggcataaatgagaacttcagactccttggacaaatagttaggggcctctatatcaaaattttctgaaaccatcactgcctctgttatgtttctctctcgtaatgaagccaactcatacggatccacataaagtcctgcaggaatgtcctgtttaattaagagacggcaggtgtgcaagtcctcaatgctttccccaaacttcactttgattaaaaggtctctgtggaaaccatctttcaaaacttcttgcctcaaaataatttcagaacacatggcccttatgccggcgtcagagcgcgcggcggtgaaggccgcggcgggcccgcgcgtgagcccggtcgccgccccgaggagcagccaggcggccgcccgaaccgccgccacccgagccgccaggacgccggaagccggacgcccgagaggggcgcgcggggccaggtgcggacgcaggaaggggcctggccgcccgcagctcctaccgcgcgctgccccagatttatcggctgggaccgagtgctgggtgcgcgcgcctagcgcccgcggttcccagct

SEQ ID NO: 10897 - RNA, 2915 nt, Homo sapiens
  source 1..2915: mol_type = other RNA
ctgaatagctgggactacaggtatgcataacctcgctgggctcgttactttgttttttttttagaggcaggatttcaccatgttgcccagggtggtctcgtactcctggattcaagcaatcctcctgcttcggcctcccaaagtgtcaggattacaggcgtgagccactgtgcccagtctcaaacaaaattaaaaattcagtttctcagtcacactagccacatttcaagtgctcagaaactttatgtggggccaggcatggtggctcatgcctgcaatcccagcactttgggaggccgaggcgggcggatcacgaggtcaggagttcgagaccagcctaaccaacatggtgaaaccctgtctctactaaaaaaatacaaaaattagccgggcgtggtggtgtgcgcctgtaatctcagctacttgggaggttgaggcgggagcattgcttgaacccgggaggcggaggatgtggtgagccgacgtcgtgccattgcactccagcctgggcaataagagcgaaactccgtctcaaaaaaaaaaaacaaaggtttatgtggccactggctactgtactggacagtacagacctagaacatgaaccaaacatcacagaaagttccagtggagaacactgctacatatctgcctgttttagttagaagccaacattttatttttattttattttattttttgagatggagtttcgctgctgttgcccaggctggagtgcaatggtgcgatctcggctcaccacaacctccgcctcccaggttcaagcaattctcctgcctcagcctcctgagtagctgggatcacaggcatgctccaccacgcccagctaattttgtatttttagtagagatggggtttctccatgttgaggctggtcttgaactcctgacctcaggtgatccacccacctcagcctcccaaagtgctgggattacaggcgtgagccactgcgccccgctaggagccaacattttaaaatagggagatttaatataaaaatccctattttagctgggcacagtagctcacacctggaatcctagcgctttgggaggccaaagcaggaagattgcttaagactaggagtttgagaccagcttgggcaccaagaccccatctctacaaaaaaaaaatttgtttaaattagctgggtatggtagcacgcacctgtagtccccaggagggtactcaggaggctgaggcaggagggtcacttggagatcacttgagccgggaggtcaaggctgttgtaagctaagatcacatcaatgcactccagcctgggcaacagtgagaccctgtctcaaaaaaaaaaaaaaaatattcccaagttcttgcttcttttgaacaactggcgtgtcaagcaactccaggccccctttaccccagggccacactggctggagccaaccagcagctggcctgttgagaggggtaatctctggtccaccagaggcccactaggcccataacacattctctccacagtagcctggcagctacctgtctttaaagccaagtgccatcctctcttcccttctccacagatgaggagtctgtggtcagagggagatgtatttttcacagatcacgcaacacacaggaagacacagcgagggtttttagattccgagaccagggtgaaaaatctgctctgatccaacaaagcacccccactgtgcttggcagccgatcagccactgtgggacgatgacccaagagtcccggacctcaccctgatgcccccatctggagactctcgggacacagcaggtgtggcgtctgggatgtactttattggacaagtggtggcccaagtcttggtctggaagcactggggccctggacccaggcactgagtttgaggaggcccagagttcagggctgtttggagcgaggccacaagcggctggtgagggagccaaggaagaggttctgcttgttggacttggagagctcggccaggcgctgctgctcctcctgctctagccggctttgccgctgtttgaaagccgccagcgggtcatcctccagggcatagtgctccagcacggttcgcacgtcctccacaccattcagtgcaatggtcttgaggaaggcagacagatccaacaagacccggtcatcagagttgccgtcccagggccgcagggcaacgccgttatagggctgcaggcggaaggcttccttcttgcagtccacaactactactcgagctgggtcccgattcagacatgaaatatcctttacatggtgtccatccatgtatcttgtggcgtcccggaataggcggtaggagatgaagccatgggggtccacactatcaatgagtggaaacgcagtcatgccagtctctgacgtaaagatgacaatttcatataaaggggcaagctgctggaacaaggtctcgatgcctgggcgcttcttaaacctccagccagtggccagcgaccactcaggatgcaagaggacgccggtgagctccaaaacgagcgtgtagggtggctggtagtacggttcctgcagagggtctgggagaaggcaagggctggtgggctcgatgatcatcattgtcgaactcatcaggaatcttggcaccattttcgtccaccgggttgtttccaaagatatagacgacgctcacagtcccaccagctccaagcagcccagcaagccagagcgcaacttttttggcatagctgggaccctctgagcccggctgctgctgtggcccttgcgccttagtgctcccgcggctcccgatctctgcggcctgatctggggcccggcggggcggcgtcgccaacctcgtgcacagtccccgcgagccgagccggagcccgcttcgcaagcgcgagaacaccgctgccgaggccgccatcttgcgctgacgccac

SEQ ID NO: 10898 - RNA, 2974 nt, Homo sapiens
  source 1..2974: mol_type = other RNA
ctgaatagctgggactacaggtatgcataacctcgctgggctcgttactttgttttttttttagaggcaggatttcaccatgttgcccagggtggtctcgtactcctggattcaagcaatcctcctgcttcggcctcccaaagtgtcaggattacaggcgtgagccactgtgcccagtctcaaacaaaattaaaaattcagtttctcagtcacactagccacatttcaagtgctcagaaactttatgtggggccaggcatggtggctcatgcctgcaatcccagcactttgggaggccgaggcgggcggatcacgaggtcaggagttcgagaccagcctaaccaacatggtgaaaccctgtctctactaaaaaaatacaaaaattagccgggcgtggtggtgtgcgcctgtaatctcagctacttgggaggttgaggcgggagcattgcttgaacccgggaggcggaggatgtggtgagccgacgtcgtgccattgcactccagcctgggcaataagagcgaaactccgtctcaaaaaaaaaaaacaaaggtttatgtggccactggctactgtactggacagtacagacctagaacatgaaccaaacatcacagaaagttccagtggagaacactgctacatatctgcctgttttagttagaagccaacattttatttttattttattttattttttgagatggagtttcgctgctgttgcccaggctggagtgcaatggtgcgatctcggctcaccacaacctccgcctcccaggttcaagcaattctcctgcctcagcctcctgagtagctgggatcacaggcatgctccaccacgcccagctaattttgtatttttagtagagatggggtttctccatgttgaggctggtcttgaactcctgacctcaggtgatccacccacctcagcctcccaaagtgctgggattacaggcgtgagccactgcgccccgctaggagccaacattttaaaatagggagatttaatataaaaatccctattttagctgggcacagtagctcacacctggaatcctagcgctttgggaggccaaagcaggaagattgcttaagactaggagtttgagaccagcttgggcaccaagaccccatctctacaaaaaaaaaatttgtttaaattagctgggtatggtagcacgcacctgtagtccccaggagggtactcaggaggctgaggcaggagggtcacttggagatcacttgagccgggaggtcaaggctgttgtaagctaagatcacatcaatgcactccagcctgggcaacagtgagaccctgtctcaaaaaaaaaaaaaaaatattcccaagttcttgcttcttttgaacaactggcgtgtcaagcaactccaggccccctttaccccagggccacactggctggagccaaccagcagctggcctgttgagaggggtaatctctggtccaccagaggcccactaggcccataacacattctctccacagtagcctggcagctacctgtctttaaagccaagtgccatcctctcttcccttctccacagatgaggagtctgtggtcagagggagatgtatttttcacagatcacgcaacacacaggaagacacagcgagggtttttagattccgagaccagggtgaaaaatctgctctgatccaacaaagcacccccactgtgcttggcagccgatcagccactgtgggacgatgacccaagagtcccggacctcaccctgatgcccccatctggagactctcgggacacagcaggtgtggcgtctgggatgtactttattggacaagtggtggcccaagtcttggtctggaagcactggggccctggacccaggcactgagtttgaggaggcccagagttcagggctgtttggagcgaggccacaagcggctggtgagggagccaaggaagaggttctgcttgttggacttggagagctcggccaggcgctgctgctcctcctgctctagccggctttgccgctgtttgaaagccgccagcgggtcatcctccagggcatagtgctccagcacggttcgcacgtcctccacaccattcagtgcaatggtcttgaggaaggcagacagatccaacaagacccggtcatcagagttgccgtcccagggccgcagggcaacgccgttatagggctgcaggcggaaggcttccttcttgcagtccacaactactactcgagctgggtcccgattcagacatgaaatatcctttacatggtgtccatccatgtatcttgtggcgtcccggaataggcggtaggagatgaagccatgggggtccacactatcaatgagtggaaacgcagtcatgccagtctctgacgtaaagatgacaatttcatataaaggggcaagctgctggaacaaggtctcgatgcctgggcgcttcttaaacctccagccagtggccagcgaccactcaggatgcaagaggacgccggtgagctccaaaacgagcgtgtagggtggctggtagtacggttcctgcagagggtctgggagaaggcaagggctggtgggctcgatgatcatctgtctataatctttgaaatatttgtatgtccggcgcaactgctgtaccagaattggatcattgtcgaactcatcaggaatcttggcaccattttcgtccaccgggttgtttccaaagatatagacgacgctcacagtcccaccagctccaagcagcccagcaagccagagcgcaacttttttggcatagctgggaccctctgagcccggctgctgctgtggcccttgcgccttagtgctcccgcggctcccgatctctgcggcctgatctggggcccggcggggcggcgtcgccaacctcgtgcacagtccccgcgagccgagccggagcccgcttcgcaagcgcgagaacaccgctgccgaggccgccatcttgcgctgacgccac

SEQ ID NO: 10899 - RNA, 1334 nt, Homo sapiens
  source 1..1334: mol_type = other RNA
ctgaatagctgggactacaggtatgcgccaccacacctggctaatttttgtattttcagtagagaagggtttcaccatgttggccaggctggtcgtgaactcctgacctcaggtgatctgcccacttcggtctaccaaagtgttggcattacggcgtgagcacctggccacgcagctgcaatcttaggcccatcattccactgagttccgaagaatatagccttttcctgaagaaactcctttcttcaatgcttcaggccagttgtgagtctctaagtaagtggacaggatatcaaacactattctgcaccatatgtggtactaaggtcttgcggggagaggcaaggacacaggctctgcttgctctcaaggacctcagcctacccttgattgatggccagtatctctgaatgatagtttttcccattctggtttctgaccatgtattcctggattggcaagcgtgcggtcttgacagagtattcccgggccttttgaaatgtcaccttcttctgaatgctttcatccacaagcccaccgaggatgtaaactttgtttagatcaacatcttcaagagcgtgttctgagtcaggagtcaggtacacaagggtttccaagggaaataaactaaagcagtcttcttctgttatgtctaacaggtaactagaaaatccatcattcatcctcacacactcttcataaaggggactgtctgttgtgaatccagtgaggcagatccaaaatggcctgtcagcttttttgtttgaaccatacaaccttcgaatctgtccagccagtctacttaattccttctttgacatgtagtgggtcatactcaaatcgatacatagtcttggtcctgagtgtttggcttccaaaagtttgtctttggttagagctctcaggaaacgtttgctgtgctgggggcaaatgcctggattttctgcacgattggcttttcttcgttctttttcttgctttcttttgctcttctttgctgcaactatcttttcccagtgtctctgttttctctggacatttttcgagcaccatgccgtactgcctgtggccaggatctctccctcctggcactcgccttccgcatcgatctgcagaagctggaagccttcaggaagtccatcttcacctgtctcctctaggatgccttcttgcccctgcagcacaggtgactctactttctgagtactcccttccaatttccagtccatggacttagtcctctgtcctttccaccagactgatatcatattgtgtccggaaatggtggattcttggtctcactgacttcaagaatgaaaccgcggaccatcgcg

SEQ ID NO: 10900 - RNA, 5428 nt, Homo sapiens
  source 1..5428: mol_type = other RNA
ctgaatagctgggactacaggtatgcgccaccacacctggctaatttttgtattttcagtagagaagggtttcaccatgttggccaggctggtcgtgaactcctgacctcaggtgatctgcccacttcggtctaccaaagtgttggcattacggcgtgagcacctggccacgcagctgcaatcttaggcccatcattccactgagttccgaagaatatagccttttcctgaagaaactcctttcttcaatgcttcaggccagttgtgagtctctaagtaagtggacaggatatcaaacactgttagagagtaaacagaaaacacagtgaccacagagggaaaaaaagaacgagtaaatgaaaaggatgttctgtaatatttcgttcaacaaacctattctgcaccatatgtggtactaaggtcttgcggggagaggcaaggacacaggctctgcttgctctcaaggacctcagcctaccctgaaagatacaggcctatgaatggatagggtgcaacagaaaggaacacagtaaaatgggaaacagaagggctctgctgtggcctgggatggggaagggccaagatgctcctgaactgaaccctgaagatcaaacaggaattcagtggtgagaggttaaaagctgggcattctagatgaaggggacaattttttttttttttttttttttttttttttttttttttgaggcggagttgcactcttgttgctcaggctggagtgcaatggcacgatctcagctcaccgcaacctgcacctcccagattcaagcaattctcttgcctcagcctccagattagctgggattacaggcgcctgccactatgccctgctaatttttgtatttttagtagagacggtgtttctccatgttggtcaggctggtctcgacctcccgacctcaggtgatctgcccacctcagcctcccaaagtgctgggattacaggtgtgagccaccgtgcccagcttttttttttgtttttgagacagagtatcactgtcacccaggctggagtgcagtggtgtgatctcggctcactgcaacctccacttcccaggttcaagtggttctcatgcctcagcctctggaataattggtattacaggcgtgcaccaccacgcctgactgatttttgtattttagtagagatggggtttcaccatgttggccaggctggtttcgaactcctaacctcaggtgatccacccacctcggcctctgaaagtggattacaggattacaggtgtgagccactgcacctggccaaggggacaatttcaactatctttaacatagttggtgacgaagaaaacagaatgcctcttagtggccagaatatatgtcatgacgtacatgcaataaagtccacacacattagtcacagaggagactgactcaaaggccacttaaacacagtgcaaagcagcagcaccagaactcacacaccctggatgggggccgtgtaagaagtaccttgattgatggccagtatctctgaatgatagtttttcccattctggtttctgaccatgtattcctggattggcaagcgtgcggtcttgacagagtattcccgggccttttgaaatgtcaccttctgtaaatatatagttaaatatttttcttataaaaattatacatgagtatattctcaatgtaatacagcattaaaaataagtagcctattgtggaatggaagaaactgcagataatgagttaactgtctcaagagcttatgtgacaatatcttactttttggggggtcactcatccacagtcctccactcactgccacttagaaccaagagggaaataagcaaaagaggcacatctgcagccacagtaggcatcaaaaggcccaagcagtctaatcaatcagagcacattctgagccctaactcagtaagacccaattctggatatctggaacttccagctcattgccaaaaggcagcatcaaattagaggaaaaggtagacaagattcaagacaggtgcaccactgcaacaagtggcattagggtgtgagaagagagagcccaattaaaagaaaggggccaggtgaagtgcctcacacaacactttgaggccaaggccagaggactgcttgagcccaggagttcaagaccagcctgagcaacatagggagatcctgtctctacaaataacaaaaaaaaaattaacagggtgtgctggtgtgtgcctgtagtcccagctactctggaggctgaagttggatgatcacttgagcctgggacatatatcaaggctgcaatgagctgtgactgcaccactgcactccagcctgggtgacagaggagaccctgtctcaaaaatataaaagggcgggctctgaaaactgcaaaaaggagtcacaagaagtccatcaacttgaggccatttagtgtcagagtacagaaactgatgtccctttataagatgttccttagtcatgaagtccctcagactgagtcatgactcagtcagattacatttgctgccttgtaagaagcacaggaaagattttctacctaagacttcaggattaaagagaaaggttcagattactgggataattaacatgccaaggcttggaaggggtctcaatagtgttaactgtatcactctaaccacccattcattgtctgttctctatgacttctccaagaggccatgtggccactcaatggacagctcttgtgacagggagttcatgcatcctgggacaacccactccagttttgatagtaccagctgataggaaattcttcttgatcttgagcaaaattctgttttctttgagacttccactcattcatcctaggtctattcccccaaggccaaaccatgcaagtaagatggcccttccaaaagatggccattcagaaacttgaaggcagtgatcatgcccctaggaatcctctagtctccagattgtagcctcagttctgtcaactcttctttgaatttcaagtcccttcatcattcaggacaagttgaacttgttctaagctagtccagtatcattttgtttacggtcccataactgactggccatcatgagtatggtctaaccaggtggaatagtgtgaagtggacctagtaccttttcggtgctgacacctgcctcacatgaaacaaaattttagatagaacttccaaaaatgttttaagcgatacagggacttatttgaaaggataaaactcctttgcatatatgagctatatgatacgtttgttttataaaaagtcttattcctttataatcactttgaagtacagaattcaaaattaggatatttgggtgttgccctagaagagcttacaatttagtttatgttctttgcacaatgattcataataaaatgactctccttgaagaaatgttgttcttagcttatttctgtgaagaagccaaactccaataacaaccaaaaagttctaaacatctcacaaatcttccagttatttttcagtttaaatgttggtggacagataatatgttaaaactgcacatctgtaagtcatgcactgctcactgaccctctgaacttaactgcctcaaaaaagggactgttggccaggcaccgtggctcatgcctgcaatctcagcactttgggagggtgaggcaggtgggtaacttcagcccagcagttcgacaccagcatgggccatacggtgaaaccccaactcaacaaaaaattagctgggcatggtagcgcccacctgtggtcccagctacttgggaagctgaggtagggggatcaattgagcctggagtaagctgattgtgccactgccctccagcctgggcagcagagcaaggccctgtcttggacggggtgggggcgctgtcaccctgctgcaggtaagactaataaacttttaattattattattgttgttttttttttttttttttagagacagggtctcactgtgttgcatcacccaggctgaagtgcagtggtgtgaccacagttctctgcagcctctaactcttgggttcaagtagtcctccagccctccagactttgtgtgtgtatgaaacagagtctcgctctgtcaccaggctggactacagtggtgtgatttcggctcactgcaacctccgcctccctggttcaagagattctcctgcctcagcctcccgagtagctgggactacaggcacatgccaccacactcagctaatttttatgtttttagtagagacagggttttcacatgttggccaggatggtatcgatctcttgaccttgtgatttgcctgacttggcctcccaaagggctgggattataggcgtgagccaccacgcccgaccctaactttttactttgaagtatttcaaacctaagaaaagttcaaaataatacaatcaatattcattcctgtaatctagactcaccagttgttaatatgttgctttttctctctgtatataaatacatattttgggctggacagggtggttcatgcctgtaatcccagtgttttgggaggctgaggcagaaggattgcttgaggcctggagttcaagaccagcctgagcaacatcaagagacttcgtctcttctgaatgctttcatccacaagcccaccgaggatgtaaactttgtttagatcaacatcttcaagagcgtgttctgagtcaggagtcaggtacacaagggtttccaagggaaataaactaaagcagtcttcttctgttatgtctaacaggtaactagaaaatccatcattcatcctcacacactcttcataaaggggactgtctgttgtgaatccagtgaggcagatccaaaatggcctgtcagcttttttgtttgaaccatacaaccttcgaatctgtccagccagtctacttaattccttctttgacatgtagtgggtcatactcaaatcgatacatagtcttggtcctgagtgtttggcttccaaaagtttgtctttggttagagctctcaggaaacgtttgctgtgctgggggcaaatgcctggattttctgcacgattggcttttcttcgttctttttcttgctttcttttgctcttctttgctgcaactatcttttcccagtgtctctgttttctctggacatttttcgagcaccatgccgtactgcctgtggccaggatctctccctcctggcactcgccttccgcatcgatctgcagaagctggaagccttcaggaagtccatcttcacctgtctcctctaggatgccttcttgcccctgcagcacaggtgactctactttctgagtactcccttccaatttccagtccatggacttagtcctctgtcctttccaccagactgatatcatattgtgtccggaaatggtggattcttggtctcactgacttcaagaatgaaaccgcggaccatcgcggtgttacaa

SEQ ID NO: 10901 - RNA, 4233 nt, Homo sapiens
  source 1..4233: mol_type = other RNA
ctgaatagctgggactacaggtatgcgccaccacacctggctaatttttgtattttcagtagagaagggtttcaccatgttggccaggctggtcgtgaactcctgacctcaggtgatctgcccacttcggtctaccaaagtgttggcattacggcgtgagcacctggccacgcagctgcaatcttaggcccatcattccactgagttccgaagaatatagccttttcctgaagaaactcctttcttcaatgcttcaggccagttgtgagtctctaagtaagtggacaggatatcaaacacttgattgatggccagtatctctgaatgatagtttttcccattctggtttctgaccatgtattcctggattggcaagcgtgcggtcttgacagagtattcccgggccttttgaaatgtcaccttctgtaaatatatagttaaatatttttcttataaaaattatacatgagtatattctcaatgtaatacagcattaaaaataagtagcctattgtggaatggaagaaactgcagataatgagttaactgtctcaagagcttatgtgacaatatcttactttttggggggtcactcatccacagtcctccactcactgccacttagaaccaagagggaaataagcaaaagaggcacatctgcagccacagtaggcatcaaaaggcccaagcagtctaatcaatcagagcacattctgagccctaactcagtaagacccaattctggatatctggaacttccagctcattgccaaaaggcagcatcaaattagaggaaaaggtagacaagattcaagacaggtgcaccactgcaacaagtggcattagggtgtgagaagagagagcccaattaaaagaaaggggccaggtgaagtgcctcacacaacactttgaggccaaggccagaggactgcttgagcccaggagttcaagaccagcctgagcaacatagggagatcctgtctctacaaataacaaaaaaaaaattaacagggtgtgctggtgtgtgcctgtagtcccagctactctggaggctgaagttggatgatcacttgagcctgggacatatatcaaggctgcaatgagctgtgactgcaccactgcactccagcctgggtgacagaggagaccctgtctcaaaaatataaaagggcgggctctgaaaactgcaaaaaggagtcacaagaagtccatcaacttgaggccatttagtgtcagagtacagaaactgatgtccctttataagatgttccttagtcatgaagtccctcagactgagtcatgactcagtcagattacatttgctgccttgtaagaagcacaggaaagattttctacctaagacttcaggattaaagagaaaggttcagattactgggataattaacatgccaaggcttggaaggggtctcaatagtgttaactgtatcactctaaccacccattcattgtctgttctctatgacttctccaagaggccatgtggccactcaatggacagctcttgtgacagggagttcatgcatcctgggacaacccactccagttttgatagtaccagctgataggaaattcttcttgatcttgagcaaaattctgttttctttgagacttccactcattcatcctaggtctattcccccaaggccaaaccatgcaagtaagatggcccttccaaaagatggccattcagaaacttgaaggcagtgatcatgcccctaggaatcctctagtctccagattgtagcctcagttctgtcaactcttctttgaatttcaagtcccttcatcattcaggacaagttgaacttgttctaagctagtccagtatcattttgtttacggtcccataactgactggccatcatgagtatggtctaaccaggtggaatagtgtgaagtggacctagtaccttttcggtgctgacacctgcctcacatgaaacaaaattttagatagaacttccaaaaatgttttaagcgatacagggacttatttgaaaggataaaactcctttgcatatatgagctatatgatacgtttgttttataaaaagtcttattcctttataatcactttgaagtacagaattcaaaattaggatatttgggtgttgccctagaagagcttacaatttagtttatgttctttgcacaatgattcataataaaatgactctccttgaagaaatgttgttcttagcttatttctgtgaagaagccaaactccaataacaaccaaaaagttctaaacatctcacaaatcttccagttatttttcagtttaaatgttggtggacagataatatgttaaaactgcacatctgtaagtcatgcactgctcactgaccctctgaacttaactgcctcaaaaaagggactgttggccaggcaccgtggctcatgcctgcaatctcagcactttgggagggtgaggcaggtgggtaacttcagcccagcagttcgacaccagcatgggccatacggtgaaaccccaactcaacaaaaaattagctgggcatggtagcgcccacctgtggtcccagctacttgggaagctgaggtagggggatcaattgagcctggagtaagctgattgtgccactgccctccagcctgggcagcagagcaaggccctgtcttggacggggtgggggcgctgtcaccctgctgcaggtaagactaataaacttttaattattattattgttgttttttttttttttttttagagacagggtctcactgtgttgcatcacccaggctgaagtgcagtggtgtgaccacagttctctgcagcctctaactcttgggttcaagtagtcctccagccctccagactttgtgtgtgtatgaaacagagtctcgctctgtcaccaggctggactacagtggtgtgatttcggctcactgcaacctccgcctccctggttcaagagattctcctgcctcagcctcccgagtagctgggactacaggcacatgccaccacactcagctaatttttatgtttttagtagagacagggttttcacatgttggccaggatggtatcgatctcttgaccttgtgatttgcctgacttggcctcccaaagggctgggattataggcgtgagccaccacgcccgaccctaactttttactttgaagtatttcaaacctaagaaaagttcaaaataatacaatcaatattcattcctgtaatctagactcaccagttgttaatatgttgctttttctctctgtatataaatacatattttgggctggacagggtggttcatgcctgtaatcccagtgttttgggaggctgaggcagaaggattgcttgaggcctggagttcaagaccagcctgagcaacatcaagagacttcgtctcttctgaatgctttcatccacaagcccaccgaggatgtaaactttgtttagatcaacatcttcaagagcgtgttctgagtcaggagtcaggtacacaagggtttccaagggaaataaactaaagcagtcttcttctgttatgtctaacaggtaactagaaaatccatcattcatcctcacacactcttcataaaggggactgtctgttgtgaatccagtgaggcagatccaaaatggcctgtcagcttttttgtttgaaccatacaaccttcgaatctgtccagccagtctacttaattccttctttgacatgtagtgggtcatactcaaatcgatacatagtcttggtcctgagtgtttggcttccaaaagtttgtctttggttagagctctcaggaaacgtttgctgtgctgggggcaaatgcctggattttctgcacgattggcttttcttcgttctttttcttgctttcttttgctcttctttgctgcaactatcttttcccagtgtctctgttttctctggacatttttcgagcaccatgccgtactgcctgtggccaggatctctccctcctggcactcgccttccgcatcgatctgcagaagctggaagccttcaggaagtccatcttcacctgtctcctctaggatgccttcttgcccctgcagcacaggtgactctactttctgagtactcccttccaatttccagtccatggacttagtcctctgtcctttccaccagactgatatcatattgtgtccggaaatggtggattcttggtctcactgacttcaagaatgaaaccgcggaccatcgcggtgttacaa

SEQ ID NO: 10902 - RNA, 1013 nt, Homo sapiens
  source 1..1013: mol_type = other RNA
ctgaatagctgggactacaggtatgcgccaccacacctggctaatttttgtattttcagtagagaagggtttcaccatgttggccaggctggtcgtgaactcctgacctcaggtgatctgcccacttcggtctaccaaagtgttggcattacggcgtgagcacctggccacgcagctgcaatcttaggcccatcattccactgagttccgaagaatatagccttttcctgaagaaactcctttcttcaatgcttcaggccagttgtgagtctctaagtaagtggacaggatatcaaacacttgattgatggccagtatctctgaatgatagtttttcccattctggtttctgaccatgtattcctggattggcaagcgtgcggtcttgacagagtattcccgggccttttgaaatgtcaccttcttctgaatgctttcatccacaagcccaccgaggatgtaaactttgtttagatcaacatcttcaagagcgtgttctgagtcaggagtcaggtacacaagggtttccaagggaaataaactaaagcagtcttcttctgttatgtctaacaggtaactagaaaatccatcattcatcctcacacactcttcataaaggggactgtctgttgtgaatccagtgaggcagatccaaaatggcctgtcagcttttttgtttgaaccatacaaccttcgaatctgtccagccagtctacttaattccgagcaccatgccgtactgcctgtggccaggatctctccctcctggcactcgccttccgcatcgatctgcagaagctggaagccttcaggaagtccatcttcacctgtctcctctaggatgccttcttgcccctgcagcacaggtgactctactttctgagtactcccttccaatttccagtccatggacttagtcctctgtcctttccaccagactgatatcatattgtgtccggaaatggtggattcttggtctcactgacttcaagaatgaaaccgcggaccatcgc

SEQ ID NO: 10903 - RNA, 983 nt, Homo sapiens
  source 1..983: mol_type = other RNA
ctgaatagctgggactacaggtatgcgccaccacacctggctaatttttgtattttcagtagagaagggtttcaccatgttggccaggctggtcgtgaactcctgacctcaggtgatctgcccacttcggtctaccaaagtgttggcattacggcgtgagcacctggccacgcagctgcaatcttaggcccatcattccactgagttccgaagaatatagccttttcctgaagaaactcctttcttcaatgcttcaggccagttgtgagtctctaagtaagtggacaggatatcaaacacttgattgatggccagtatctctgaatgatagtttttcccattctggtttctgaccatgtattcctggattggcaagcgtgcggtcttgacagagtattcccgggccttttgaaatgtcaccttcttctgaatgctttcatccacaagcccaccgaggatgtaaactttgtttagatcaacatcttcaagagcgtgttctgagtcaggagtcaggtacacaagggtttccaagggaaataaactaaagcagtcttcttctgttatgtctaacaggtaactagaaaatccatcattcatcctcacacactcttcataaaggggactgtctgttgtgaatccagtgaggcagatccaaaatggcctgtcagcttttttgtttgaaccatacaaccttcgaatctgtccagccagtctacttaattccgagcaccatgccgtactgcctgtggccaggatctctccctcctggcactcgccttccgcatcgatctgcagaagctggaagccttcaggaagtccatcttcacctgtctcctctaggatgccttcttgcccctgcagcacaggtgactctactttctgagtactcccttccaatttccagtccatggacttagtcctctgtcctttccaccagactgatcccctcacccccacgcagcggcagcggcgcgcatcggatc

SEQ ID NO: 10904 - RNA, 1111 nt, Homo sapiens
  source 1..1111: mol_type = other RNA
ctgaatagctgggactacaggtatgcgccaccacacctggctaatttttgtattttcagtagagaagggtttcaccatgttggccaggctggtcgtgaactcctgacctcaggtgatctgcccacttcggtctaccaaagtgttggcattacggcgtgagcacctggccacgcagctgcaatcttaggcccatcattccactgagttccgaagaatatagccttttcctgaagaaactcctttcttcaatgcttcaggccagttgtgagtctctaagtaagtggacaggatatcaaacacttgattgatggccagtatctctgaatgatagtttttcccattctggtttctgaccatgtattcctggattggcaagcgtgcggtcttgacagagtattcccgggccttttgaaatgtcaccttcttctgaatgctttcatccacaagcccaccgaggatgtaaactttgtttagatcaacatcttcaagagcgtgttctgagtcaggagtcaggtacacaagggtttccaagggaaataaactaaagcagtcttcttctgttatgtctaacaggtaactagaaaatccatcattcatcctcacacactcttcataaaggggactgtctgttgtgaatccagtgaggcagatccaaaatggcctgtcagcttttttgtttgaaccatacaaccttcgaatctgtccagccagtctacttaattccttctttgacatgtagtgggtcatactcaaatcgatacatagtcttggtcctgagtgtttggcttccaaaagtttgtctttggttagagctctcaggaaacgtttgctgtgctgggggcaaatgccgagcaccatgccgtactgcctgtggccaggatctctccctcctggcactcgccttccgcatcgatctgcagaagctggaagccttcaggaagtccatcttcacctgtctcctctaggatgccttcttgcccctgcagcacaggtgactctactttctgagtactcccttccaatttccagtccatggacttagtcctctgtcctttccaccagactgatcccctcacccccacgcagcggcagcggcgcgcatcggatcccc

SEQ ID NO: 10905 - RNA, 1245 nt, Homo sapiens
  source 1..1245: mol_type = other RNA
ctgaatagctgggactacaggtatgcgccaccacacctggctaatttttgtattttcagtagagaagggtttcaccatgttggccaggctggtcgtgaactcctgacctcaggtgatctgcccacttcggtctaccaaagtgttggcattacggcgtgagcacctggccacgcagctgcaatcttaggcccatcattccactgagttccgaagaatatagccttttcctgaagaaactcctttcttcaatgcttcaggccagttgtgagtctctaagtaagtggacaggatatcaaacacttgattgatggccagtatctctgaatgatagtttttcccattctggtttctgaccatgtattcctggattggcaagcgtgcggtcttgacagagtattcccgggccttttgaaatgtcaccttcttctgaatgctttcatccacaagcccaccgaggatgtaaactttgtttagatcaacatcttcaagagcgtgttctgagtcaggagtcaggtacacaagggtttccaagggaaataaactaaagcagtcttcttctgttatgtctaacaggtaactagaaaatccatcattcatcctcacacactcttcataaaggggactgtctgttgtgaatccagtgaggcagatccaaaatggcctgtcagcttttttgtttgaaccatacaaccttcgaatctgtccagccagtctacttaattccttctttgacatgtagtgggtcatactcaaatcgatacatagtcttggtcctgagtgtttggcttccaaaagtttgtctttggttagagctctcaggaaacgtttgctgtgctgggggcaaatgcctggattttctgcacgattggcttttcttcgttctttttcttgctttcttttgctcttctttgctgcaactatcttttcccagtgtctctgttttctctggacatttttcgagcaccatgccgtactgcctgtggccaggatctctccctcctggcactcgccttccgcatcgatctgcagaagctggaagccttcaggaagtccatcttcacctgtctcctctaggatgccttcttgcccctgcagcacaggtgactctactttctgagtactcccttccaatttccagtccatggacttagtcctctgtcctttccaccagactgatatcatattgtgtccggaaatggtggattcttggtctcactgacttcaagaatgaaaccgcggaccatc

SEQ ID NO: 10906 - RNA, 1220 nt, Homo sapiens
  source 1..1220: mol_type = other RNA
ctgaatagctgggactacaggtatgcgccaccacacctggctaatttttgtattttcagtagagaagggtttcaccatgttggccaggctggtcgtgaactcctgacctcaggtgatctgcccacttcggtctaccaaagtgttggcattacggcgtgagcacctggccacgcagctgcaatcttaggcccatcattccactgagttccgaagaatatagccttttcctgaagaaactcctttcttcaatgcttcaggccagttgtgagtctctaagtaagtggacaggatatcaaacacttgattgatggccagtatctctgaatgatagtttttcccattctggtttctgaccatgtattcctggattggcaagcgtgcggtcttgacagagtattcccgggccttttgaaatgtcaccttcttctgaatgctttcatccacaagcccaccgaggatgtaaactttgtttagatcaacatcttcaagagcgtgttctgagtcaggagtcaggtacacaagggtttccaagggaaataaactaaagcagtcttcttctgttatgtctaacaggtaactagaaaatccatcattcatcctcacacactcttcataaaggggactgtctgttgtgaatccagtgaggcagatccaaaatggcctgtcagcttttttgtttgaaccatacaaccttcgaatctgtccagccagtctacttaattccttctttgacatgtagtgggtcatactcaaatcgatacatagtcttggtcctgagtgtttggcttccaaaagtttgtctttggttagagctctcaggaaacgtttgctgtgctgggggcaaatgcctggattttctgcacgattggcttttcttcgttctttttcttgctttcttttgctcttctttgctgcaactatcttttcccagtgtctctgttttctctggacatttttcgagcaccatgccgtactgcctgtggccaggatctctccctcctggcactcgccttccgcatcgatctgcagaagctggaagccttcaggaagtccatcttcacctgtctcctctaggatgccttcttgcccctgcagcacaggtgactctactttctgagtactcccttccaatttccagtccatggacttagtcctctgtcctttccaccagactgatcccctcacccccacgcagcggcagcggcgcgcatcggatcccc

SEQ ID NO: 10907 - RNA, 1253 nt, Homo sapiens
  source 1..1253: mol_type = other RNA
ctgaatagctgggactacaggtatgcgccaccacacctggctaatttttgtattttcagtagagaagggtttcaccatgttggccaggctggtcgtgaactcctgacctcaggtgatctgcccacttcggtctaccaaagtgttggcattacggcgtgagcacctggccacgcagctgcaatcttaggcccatcattccactgagttccgaagaatatagccttttcctgaagaaactcctttcttcaatgcttcaggccagttgtgagtctctaagtaagtggacaggatatcaaacacttgattgatggccagtatctctgaatgatagtttttcccattctggtttctgaccatgtattcctggattggcaagcgtgcggtcttgacagagtattcccgggccttttgaaatgtcaccttcttctgaatgctttcatccacaagcccaccgaggatgtaaactttgtttagatcaacatcttcaagagcgtgttctgagtcaggagtcaggtacacaagggtttccaagggaaataaactaaagcagtcttcttctgttatgtctaacaggtaactagaaaatccatcattcatcctcacacactcttcataaaggggactgtctgttgtgaatccagtgaggcagatccaaaatggcctgtcagcttttttgtttgaaccatacaaccttcgaatctgtccagccagtctacttaattccttctttgacatgtagtgggtcatactcaaatcgatacatagtcttggtcctgagtgtttggcttccaaaagtttgtctttggttagagctctcaggaaacgtttgctgtgctgggggcaaatgcctggattttctgcacgattggcttttcttcgttctttttcttgctttcttttgctcttctttgctgcaactatcttttcccagtgtctctgttttctctggacatttttcttatattatccagaaaacaaaattgtttgagaacgagcaccatgccgtactgcctgtggccaggatctctccctcctggcactcgccttccgcatcgatctgcagaagctggaagccttcaggaagtccatcttcacctgtctcctctaggatgccttcttgcccctgcagcacaggtgactctactttctgagtactcccttccaatttccagtccatggacttagtcctctgtcctttccaccagactgatcccctcacccccacgcagcggcagcggcgcgcatcggatccc

SEQ ID NO: 10908 - RNA, 1367 nt, Homo sapiens
  source 1..1367: mol_type = other RNA
ctgaatagctgggactacaggtatgcgccaccacacctggctaatttttgtattttcagtagagaagggtttcaccatgttggccaggctggtcgtgaactcctgacctcaggtgatctgcccacttcggtctaccaaagtgttggcattacggcgtgagcacctggccacgcagctgcaatcttaggcccatcattccactgagttccgaagaatatagccttttcctgaagaaactcctttcttcaatgcttcaggccagttgtgagtctctaagtaagtggacaggatatcaaacacttgattgatggccagtatctctgaatgatagtttttcccattctggtttctgaccatgtattcctggattggcaagcgtgcggtcttgacagagtattcccgggccttttgaaatgtcaccttcttctgaatgctttcatccacaagcccaccgaggatgtaaactttgtttagatcaacatcttcaagagcgtgttctgagtcaggagtcaggtacacaagggtttccaagggaaataaactaaagcagtcttcttctgttatgtctaacaggtaactagaaaatccatcattcatcctcacacactcttcataaaggggactgtctgttgtgaatccagtgaggcagatccaaaatggcctgtcagcttttttgtttgaaccatacaaccttcgaatctgtccagccagtctacttaattctagtttactaaggaatcccagaagctggagttgaccatattcttcggaaagctgtacccttctgggcctccctcatggcgagcaggaattccaggcttagtggatgttctaccttctttgacatgtagtgggtcatactcaaatcgatacatagtcttggtcctgagtgtttggcttccaaaagtttgtctttggttagagctctcaggaaacgtttgctgtgctgggggcaaatgcctggattttctgcacgattggcttttcttcgttctttttcttgctttcttttgctcttctttgctgcaactatcttttcccagtgtctctgttttctctggacatttttcgagcaccatgccgtactgcctgtggccaggatctctccctcctggcactcgccttccgcatcgatctgcagaagctggaagccttcaggaagtccatcttcacctgtctcctctaggatgccttcttgcccctgcagcacaggtgactctactttctgagtactcccttccaatttccagtccatggacttagtcctctgtcctttccaccagactgatatcatattgtgtccggaaatggtggattcttggtctcactgacttcaagaatgaaaccgcggaccatcgcggtgttac

SEQ ID NO: 10909 - RNA, 1332 nt, Homo sapiens
  source 1..1332: mol_type = other RNA
ctgaatagctgggactacaggtatgcgccaccacacctggctaatttttgtattttcagtagagaagggtttcaccatgttggccaggctggtcgtgaactcctgacctcaggtgatctgcccacttcggtctaccaaagtgttggcattacggcgtgagcacctggccacgcagctgcaatcttaggcccatcattccactgagttccgaagaatatagccttttcctgaagaaactcctttcttcaatgcttcaggccagttgtgagtctctaagtaagtggacaggatatcaaacacttgattgatggccagtatctctgaatgatagtttttcccattctggtttctgaccatgtattcctggattggcaagcgtgcggtcttgacagagtattcccgggccttttgaaatgtcaccttcttctgaatgctttcatccacaagcccaccgaggatgtaaactttgtttagatcaacatcttcaagagcgtgttctgagtcaggagtcaggtacacaagggtttccaagggaaataaactaaagcagtcttcttctgttatgtctaacaggtaactagaaaatccatcattcatcctcacacactcttcataaaggggactgtctgttgtgaatccagtgaggcagatccaaaatggcctgtcagcttttttgtttgaaccatacaaccttcgaatctgtccagccagtctacttaattctagtttactaaggaatcccagaagctggagttgaccatattcttcggaaagctgtacccttctgggcctccctcatggcgagcaggaattccaggcttagtggatgttctaccttctttgacatgtagtgggtcatactcaaatcgatacatagtcttggtcctgagtgtttggcttccaaaagtttgtctttggttagagctctcaggaaacgtttgctgtgctgggggcaaatgcctggattttctgcacgattggcttttcttcgttctttttcttgctttcttttgctcttctttgctgcaactatcttttcccagtgtctctgttttctctggacatttttcgagcaccatgccgtactgcctgtggccaggatctctccctcctggcactcgccttccgcatcgatctgcagaagctggaagccttcaggaagtccatcttcacctgtctcctctaggatgccttcttgcccctgcagcacaggtgactctactttctgagtactcccttccaatttccagtccatggacttagtcctctgtcctttccaccagactgatcccctcacccccacgcagcggcagcggcgcgcatcggatcccc

SEQ ID NO: 10910 - RNA, 948 nt, Homo sapiens
  source 1..948: mol_type = other RNA
ctgaatagctgggactacaggtatgcgccaccacacctggctaatttttgtattttcagtagagaagggtttcaccatgttggccaggctggtcgtgaactcctgacctcaggtgatctgcccacttcggtctaccaaagtgttggcattacggcgtgagcacctggccacgcagctgcaatcttaggcccatcattccactgagttccgaagaatatagccttttcctgaagaaactcctttcttcaatgcttcaggccagttgtgagtctcttgattgatggccagtatctctgaatgatagtttttcccattctggtttctgaccatgtattcctggattggcaagcgtgcggtcttgacagagtattcccgggccttttgaaatgtcaccttcttctgaatgctttcatccacaagcccaccgaggatgtaaactttgtttagatcaacatcttcaagagcgtgttctgagtcaggagtcaggtacacaagggtttccaagggaaataaactaaagcagtcttcttctgttatgtctaacaggtaactagaaaatccatcattcatcctcacacactcttcataaaggggactgtctgttgtgaatccagtgaggcagatccaaaatggcctgtcagcttttttgtttgaaccatacaaccttcgaatctgtccagccagtcgagcaccatgccgtactgcctgtggccaggatctctccctcctggcactcgccttccgcatcgatctgcagaagctggaagccttcaggaagtccatcttcacctgtctcctctaggatgccttcttgcccctgcagcacaggtgactctactttctgagtactcccttccaatttccagtccatggacttagtcctctgtcctttccaccagactgatcccctcacccccacgcagcggcagcggcgcgcatcggatcccc

SEQ ID NO: 10911 - RNA, 993 nt, Homo sapiens
  source 1..993: mol_type = other RNA
ctgaatagctgggactacaggtatgcgccaccacacctggctaatttttgtattttcagtagagaagggtttcaccatgttggccaggctggtcgtgaactcctgacctcaggtgatctgcccacttcggtctaccaaagtgttggcattacggcgtgagcacctggccacgcagctgcaatcttaggcccatcattccactgagttccgaagaatatagccttttcctgaagaaactcctttcttcaatgcttcaggccagttgtgagtctcttgattgatggccagtatctctgaatgatagtttttcccattctggtttctgaccatgtattcctggattggcaagcgtgcggtcttgacagagtattcccgggccttttgaaatgtcaccttcttctgaatgctttcatccacaagcccaccgaggatgtaaactttgtttagatcaacatcttcaagagcgtgttctgagtcaggagtcaggtacacaagggtttccaagggaaataaactaaagcagtcttcttctgttatgtctaacaggtaactagaaaatccatcattcatcctcacacactcttcataaaggggactgtctgttgtgaatccagtgaggcagatccaaaatggcctgtcagcttttttgtttgaaccatacaaccttcgaatctgtccagccagtctacttaattccgagcaccatgccgtactgcctgtggccaggatctctccctcctggcactcgccttccgcatcgatctgcagaagctggaagccttcaggaagtccatcttcacctgtctcctctaggatgccttcttgcccctgcagcacaggtgactctactttctgagtactcccttccaatttccagtccatggacttagtcctctgtcctttccaccagactgatatcatattgtgtccggaaatggtggattcttggtctcactgacttcaagaatgaaaccgcggaccatcgcggtgtta

SEQ ID NO: 10912 - RNA, 959 nt, Homo sapiens
  source 1..959: mol_type = other RNA
ctgaatagctgggactacaggtatgcgccaccacacctggctaatttttgtattttcagtagagaagggtttcaccatgttggccaggctggtcgtgaactcctgacctcaggtgatctgcccacttcggtctaccaaagtgttggcattacggcgtgagcacctggccacgcagctgcaatcttaggcccatcattccactgagttccgaagaatatagccttttcctgaagaaactcctttcttcaatgcttcaggccagttgtgagtctcttgattgatggccagtatctctgaatgatagtttttcccattctggtttctgaccatgtattcctggattggcaagcgtgcggtcttgacagagtattcccgggccttttgaaatgtcaccttcttctgaatgctttcatccacaagcccaccgaggatgtaaactttgtttagatcaacatcttcaagagcgtgttctgagtcaggagtcaggtacacaagggtttccaagggaaataaactaaagcagtcttcttctgttatgtctaacaggtaactagaaaatccatcattcatcctcacacactcttcataaaggggactgtctgttgtgaatccagtgaggcagatccaaaatggcctgtcagcttttttgtttgaaccatacaaccttcgaatctgtccagccagtctacttaattccgagcaccatgccgtactgcctgtggccaggatctctccctcctggcactcgccttccgcatcgatctgcagaagctggaagccttcaggaagtccatcttcacctgtctcctctaggatgccttcttgcccctgcagcacaggtgactctactttctgagtactcccttccaatttccagtccatggacttagtcctctgtcctttccaccagactgatcccctcacccccacgcagcggcagcggcgcgcatcggatcccc

SEQ ID NO: 10913 - RNA, 1223 nt, Homo sapiens
  source 1..1223: mol_type = other RNA
ctgaatagctgggactacaggtatgcgccaccacacctggctaatttttgtattttcagtagagaagggtttcaccatgttggccaggctggtcgtgaactcctgacctcaggtgatctgcccacttcggtctaccaaagtgttggcattacggcgtgagcacctggccacgcagctgcaatcttaggcccatcattccactgagttccgaagaatatagccttttcctgaagaaactcctttcttcaatgcttcaggccagttgtgagtctcttgattgatggccagtatctctgaatgatagtttttcccattctggtttctgaccatgtattcctggattggcaagcgtgcggtcttgacagagtattcccgggccttttgaaatgtcaccttcttctgaatgctttcatccacaagcccaccgaggatgtaaactttgtttagatcaacatcttcaagagcgtgttctgagtcaggagtcaggtacacaagggtttccaagggaaataaactaaagcagtcttcttctgttatgtctaacaggtaactagaaaatccatcattcatcctcacacactcttcataaaggggactgtctgttgtgaatccagtgaggcagatccaaaatggcctgtcagcttttttgtttgaaccatacaaccttcgaatctgtccagccagtctacttaattccttctttgacatgtagtgggtcatactcaaatcgatacatagtcttggtcctgagtgtttggcttccaaaagtttgtctttggttagagctctcaggaaacgtttgctgtgctgggggcaaatgcctggattttctgcacgattggcttttcttcgttctttttcttgctttcttttgctcttctttgctgcaactatcttttcccagtgtctctgttttctctggacatttttcgagcaccatgccgtactgcctgtggccaggatctctccctcctggcactcgccttccgcatcgatctgcagaagctggaagccttcaggaagtccatcttcacctgtctcctctaggatgccttcttgcccctgcagcacaggtgactctactttctgagtactcccttccaatttccagtccatggacttagtcctctgtcctttccaccagactgatatcatattgtgtccggaaatggtggattcttggtctcactgacttcaagaatgaaaccgcggaccatcgcggt

SEQ ID NO: 10914 - RNA, 1193 nt, Homo sapiens
  source 1..1193: mol_type = other RNA
ctgaatagctgggactacaggtatgcgccaccacacctggctaatttttgtattttcagtagagaagggtttcaccatgttggccaggctggtcgtgaactcctgacctcaggtgatctgcccacttcggtctaccaaagtgttggcattacggcgtgagcacctggccacgcagctgcaatcttaggcccatcattccactgagttccgaagaatatagccttttcctgaagaaactcctttcttcaatgcttcaggccagttgtgagtctcttgattgatggccagtatctctgaatgatagtttttcccattctggtttctgaccatgtattcctggattggcaagcgtgcggtcttgacagagtattcccgggccttttgaaatgtcaccttcttctgaatgctttcatccacaagcccaccgaggatgtaaactttgtttagatcaacatcttcaagagcgtgttctgagtcaggagtcaggtacacaagggtttccaagggaaataaactaaagcagtcttcttctgttatgtctaacaggtaactagaaaatccatcattcatcctcacacactcttcataaaggggactgtctgttgtgaatccagtgaggcagatccaaaatggcctgtcagcttttttgtttgaaccatacaaccttcgaatctgtccagccagtctacttaattccttctttgacatgtagtgggtcatactcaaatcgatacatagtcttggtcctgagtgtttggcttccaaaagtttgtctttggttagagctctcaggaaacgtttgctgtgctgggggcaaatgcctggattttctgcacgattggcttttcttcgttctttttcttgctttcttttgctcttctttgctgcaactatcttttcccagtgtctctgttttctctggacatttttcgagcaccatgccgtactgcctgtggccaggatctctccctcctggcactcgccttccgcatcgatctgcagaagctggaagccttcaggaagtccatcttcacctgtctcctctaggatgccttcttgcccctgcagcacaggtgactctactttctgagtactcccttccaatttccagtccatggacttagtcctctgtcctttccaccagactgatcccctcacccccacgcagcggcagcggcgcgcatcggatcccc

SEQ ID NO: 10915 - RNA, 1040 nt, Homo sapiens
  source 1..1040: mol_type = other RNA
ctgaatagctgggactacaggtatgcgccaccacacctggctaatttttgtattttcagtagagaagggtttcaccatgttggccaggctggtcgtgaactcctgacctcaggtgatctgcccacttcggtctaccaaagtgttggcattacggcgtgagcacctggccacgcagctgcaatcttaggcccatcattccactgagttccgaagaatatagccttttcctgaagaaactcctttcttcaatgcttcaggccagttgtgagtctcttgattgatggccagtatctctgaatgatagtttttcccattctggtttctgaccatgtattcctggattggcaagcgtgcggtcttgacagagtattcccgggccttttgaaatgtcaccttcttctgaatgctttcatccacaagcccaccgaggatgtaaactttgtttagatcaacatcttcaagagcgtgttctgagtcaggagtcaggtacacaagggtttccaagggaaataaactaaagcagtcttcttctgttatgtctaacttctttgacatgtagtgggtcatactcaaatcgatacatagtcttggtcctgagtgtttggcttccaaaagtttgtctttggttagagctctcaggaaacgtttgctgtgctgggggcaaatgcctggattttctgcacgattggcttttcttcgttctttttcttgctttcttttgctcttctttgctgcaactatcttttcccagtgtctctgttttctctggacatttttcgagcaccatgccgtactgcctgtggccaggatctctccctcctggcactcgccttccgcatcgatctgcagaagctggaagccttcaggaagtccatcttcacctgtctcctctaggatgccttcttgcccctgcagcacaggtgactctactttctgagtactcccttccaatttccagtccatggacttagtcctctgtcctttccaccagactgatcccctcacccccacgcagcggcagcggcgcgcatcggatcccc

SEQ ID NO: 10916 - RNA, 1036 nt, Homo sapiens
  source 1..1036: mol_type = other RNA
ctgaatagctgggactacaggtatgcgccaccacacctggctaatttttgtattttcagtagagaagggtttcaccatgttggccaggctggtcgtgaactcctgacctcaggtgatctgcccacttcggtctaccaaagtgttggcattacggcgtgagcacctggccacgcagctgcaatcttaggcccatcattccactgagttccgaagaatatagccttttcctgaagaaactcctttcttcaatgcttcaggccagttgtgagtctcttgattgatggccagtatctctgaatgatagtttttcccattctggtttctgaccatgtattcctggattggcaagcgtgcggtcttgacagagtattcccgggccttttgaaatgtcaccttcttctgaatgctttcatccacaagcccaccgaggatgtaaactttgtttagatcaacatcttcaagagcgtgttctgagtcaggagtcaggtacacaagggtttccaagggaaataaactaaagcagtcttcttctgttatgtcttctttgacatgtagtgggtcatactcaaatcgatacatagtcttggtcctgagtgtttggcttccaaaagtttgtctttggttagagctctcaggaaacgtttgctgtgctgggggcaaatgcctggattttctgcacgattggcttttcttcgttctttttcttgctttcttttgctcttctttgctgcaactatcttttcccagtgtctctgttttctctggacatttttcgagcaccatgccgtactgcctgtggccaggatctctccctcctggcactcgccttccgcatcgatctgcagaagctggaagccttcaggaagtccatcttcacctgtctcctctaggatgccttcttgcccctgcagcacaggtgactctactttctgagtactcccttccaatttccagtccatggacttagtcctctgtcctttccaccagactgatcccctcacccccacgcagcggcagcggcgcgcatcggatcccc

SEQ ID NO: 10917 - RNA, 3343 nt, Homo sapiens
  source 1..3343: mol_type = other RNA
ctgaatagctgggactacaggtatgtaccaccacacccagctaattttttttgtagagatggggtttagccatgttgcccaggctggtcttgaactcctgggcttaagcaatccacccaccttggccccccaaagtgctgtgattacatgtgtgagccactgtgtccagtcgacagtagcctttttactgtgatgtcaataaaccaacatctgaagatgacaggaactggattcagagtctgtgtaaattttctcaatgagtgaccgagcatgtaaatttaactcaaatgaaattactacaataattgctttaaaaacatatttaggaaaatgaggtgaccctagatgagcttatttatatgtctcctctaacagaaatcacctcatggtaagagttgcttcttttggctcagttcacctgagaacaacttcatttggaacttttcttagccatttaacgtaacaggagactgactcaaagttggttctagtggatgaagcaaaatagacatgaccagcatggccaatcaatgagcttcattcaacggagcgtcctggccaagtgccacagccacgctggccagacacactgaccagttacgcatttcccaccagccaaatgccactgtttactaaaccatgatttcagtaggaaaaagagctctggaatcaaggccctcactgcagtacctgggtggggtgtccatggcctggcctgtagtaaaccctctgccttccactgtgttcacgttcgcagctctggcactggggcatctggcacttttttaaaagagatgtctctgcctctagatgaacaatctggaacttcagaatacagatcaaagaatgaagcagatctttcagtggcctcatcctgtggcacctgcccagccatttaactcccctgtcctcccaccctacataaagtgtttcccacaccagagtgtgcacaacatggtgactccaaatcccaaggaagttgagtttagctggaggttaaccccgtgctcagaaacccatctgttatctttccagcttcaggtttcagagcagtttataaatggcataatacaagggtaatgtgagtaaaatctgagagttttgttcattatcaagttatccacacagtgcccaattaagtaaggtgatctagtggagtaatacttctggcctgggagaaaaataaaaccagtcaaatcacacctttctctaaaatgtcccattaaaaaaatatggaataggccgggcgcggtggctcacgcctgtaatcccagcactctgggaggccaaggtgggcggatcacgaggtcaggagatcgagaccatcctggctaacacagtgaaaccccatctctactaaaaatacaaaaaaattagctgggcgcggtggcaggtgcctgtagtcccagctactcgggaggctgaggcaggagagtggcgtgaatccaggaggtggagtttgcagtgagctgagaatgtgccactacactccagcctgggcgacagagtgaaactccatctcaaaaaaaaaaaaaattatatgtatgtgtgtatgtatatatatgtatatatatatatatatgtatgtatgtatgtgtgtgtgtgtgtgtgtgtgtgtgtgtgtatatatggaataaagtttgagattccctgctttttcatgttaccttagcctcaattttaaacttacattgtttgttaaaattatcaaatggacaacctcattgctatggaacaaaaaagactgtgaggaaaaagaatcataacttggaaaaaaataagtgaaaaggcattgagagattgctaagatttgttaagttaaaacaataatatatctagaaaagactgtgaaaatatatatctcaaaagagaacaaggcatagtcagaaggctcagtaaaacaattactttaaaagctgactaataaaaagggtaagtgaaagaactcttccatccttgacccttcctcacttcctccctccgactccaccagtctggatgcactaaagcagaataacctaaaagccatgaaaaagtgctggtatttttcaggatctcttcaagacaccttccgtcttggtaacctgaattctctctctgatcaaggcagctgatggactttcaatgtatttggagatgccggttcaaaaacgtcatcatcatcttctgctccttcttctatcggtttcatcttggcagaggctcgctggtgtggggatgacacatgaagagaggacatgctggaggtaccccgaagaaactggtgcaagccgtcgtcactgtcactggagctggctatactgttcctcatttccaacatggagatctgtgtgcagaggctgagctgatgttccagctttttggcttttttatcatttaaggtgggatcattcaatgagtagagcttatttgtgatgtcttttccaataagatacctaaagatttcatacaagaaaggttctgattccagaaagtatgttaatctttctcttgaccagcataaaaatctgcagttatcatctgcaataatggtgacctggaatttttcacctttgtgcatctgagttgatctaaattcaggagaatctataaaggcacaggggtaaatgttatgcagaaaatgtcctcgataggagaccttcatttttcccttcaagagaatactcagacggtcatcaactgaggttttatcctctgcagcataagtttggccctttttcaaggtttggatcatgcaaaactgtccagttagtcttctgaacaaatctggaggcacacggagtggttcaaacaatcgccggtacatgccactgagttccttttcaatctttaccggtctcttcttgtataaaagatacgacagatgcaaaatgttgacacccaagaacacagagttccagatcattatatccaaggcacatcggtagagagtggcccagacgatataaagggtacatcctagagttaacattcccctaagaaatatcatatgaaggtgaagagtagttggaataaccaacccaactgcaaaacaaatatttgctacatgaaaaaccagatgatgtatctctctccagttttcacaagtggtcttattggaaggcacaggtatgatactttctaactcaggtgtaaaacctatggcagttgattctctcaatgggctggactctgtataattcattttgaaaattcattgctaagagtcttttcgcacttattcatgcttcaaagcaggcagtttctgggacttgtctggccaacaacccgttcccaaaggctcggggaaggaggttgcgggtgggtggcgcggacctcgggtccccagccatcggcgctctcc

SEQ ID NO: 10918 - RNA, 3271 nt, Homo sapiens
  source 1..3271: mol_type = other RNA
ctgaatagctgggactacaggtatgtaccaccacacccagctaattttttttgtagagatggggtttagccatgttgcccaggctggtcttgaactcctgggcttaagcaatccacccaccttggccccccaaagtgctgtgattacatgtgtgagccactgtgtccagtcgacagtagcctttttactgtgatgtcaataaaccaacatctgaagatgacaggaactggattcagagtctgtgtaaattttctcaatgagtgaccgagcatgtaaatttaactcaaatgaaattactacaataattgctttaaaaacatatttaggaaaatgaggtgaccctagatgagcttatttatatgtctcctctaacagaaatcacctcatggtaagagttgcttcttttggctcagttcacctgagaacaacttcatttggaacttttcttagccatttaacgtaacaggagactgactcaaagttggttctagtggatgaagcaaaatagacatgaccagcatggccaatcaatgagcttcattcaacggagcgtcctggccaagtgccacagccacgctggccagacacactgaccagttacgcatttcccaccagccaaatgccactgtttactaaaccatgatttcagtaggaaaaagagctctggaatcaaggccctcactgcagtacctgggtggggtgtccatggcctggcctgtagtaaaccctctgccttccactgtgttcacgttcgcagctctggcactggggcatctggcacttttttaaaagagatgtctctgcctctagatgaacaatctggaacttcagaatacagatcaaagaatgaagcagatctttcagtggcctcatcctgtggcacctgcccagccatttaactcccctgtcctcccaccctacataaagtgtttcccacaccagagtgtgcacaacatggtgactccaaatcccaaggaagttgagtttagctggaggttaaccccgtgctcagaaacccatctgttatctttccagcttcaggtttcagagcagtttataaatggcataatacaagggtaatgtgagtaaaatctgagagttttgttcattatcaagttatccacacagtgcccaattaagtaaggtgatctagtggagtaatacttctggcctgggagaaaaataaaaccagtcaaatcacacctttctctaaaatgtcccattaaaaaaatatggaataggccgggcgcggtggctcacgcctgtaatcccagcactctgggaggccaaggtgggcggatcacgaggtcaggagatcgagaccatcctggctaacacagtgaaaccccatctctactaaaaatacaaaaaaattagctgggcgcggtggcaggtgcctgtagtcccagctactcgggaggctgaggcaggagagtggcgtgaatccaggaggtggagtttgcagtgagctgagaatgtgccactacactccagcctgggcgacagagtgaaactccatctcaaaaaaaaaaaaaattatatgtatgtgtgtatgtatatatatgtatatatatatatatatgtatgtatgtatgtgtgtgtgtgtgtgtgtgtgtgtgtgtgtatatatggaataaagtttgagattccctgctttttcatgttaccttagcctcaattttaaacttacattgtttgttaaaattatcaaatggacaacctcattgctatggaacaaaaaagactgtgaggaaaaagaatcataacttggaaaaaaataagtgaaaaggcattgagagattgctaagatttgttaagttaaaacaataatatatctagaaaagactgtgaaaatatatatctcaaaagagaacaaggcatagtcagaaggctcagtaaaacaattactttaaaagctgactaataaaaagggtaagtgaaagaactcttccatccttgacccttcctcacttcctccctccgactccaccagtctggatgcactaaagcagaataacctaaaagccatgaaaaagtgctggtatttttcaggatctcttcaagacaccttccgtcttggtaacctgaattctctctctgatcaaggcagctgatggactttcaatgtatttggagatgccggttcaaaaacgtcatcatcatcttctgctccttcttctatcggtttcatcttggcagaggctcgctggtgtggggatgacacatgaagagaggacatgctggaggtaccccgaagaaactggtgcaagccgtcgtcactgtcactggagctggctatactgttcctcatttccaacatggagatctgtgtgcagaggctgagctgatgttccagctttttggcttttttatcatttaaggtgggatcattcaatgagtagagcttatttgtgatgtcttttccaataagatacctaaagatttcatacaagaaaggttctgattccagaaagtatgttaatctttctcttgaccagcataaaaatctgcagttatcatctgcaataatggtgacctggaatttttcacctttgtgcatctgagttgatctaaattcaggagaatctataaaggcacaggggtaaatgttatgcagaaaatgtcctcgataggagaccttcatttttcccttcaagagaatactcagacggtcatcaactgaggttttatcctctgcagcataagtttggccctttttcaaggtttggatcatgcaaaactgtccagttagtcttctgaacaaatctggaggcacacggagtggttcaaacaatcgccggtacatgccactgagttccttttcaatctttaccggtctcttcttgtataaaagatacgacagatgcaaaatgttgacacccaagaacacagagttccagatcattatatccaaggcacatcggtagagagtggcccagacgatataaagggtacatcctagagttaacattcccctaagaaatatcatatgaaggtgaagagtagttggaataaccaacccaactgcaaaacaaatatttgctacatgaaaaaccagatgatgtatctctctccagttttcacaagtggtcttattggaaggcacaggtatgatactttctaactcaggtgtaaaacctatggcagttgattctctcaatgggctggactctgtataattcattttgaaaattccaaggggcttgccgccgcagagcgcgggagccggcactcggtggggccgagggcccggggacgctggggctgcctg

SEQ ID NO: 10919 - RNA, 3384 nt, Homo sapiens
  source 1..3384: mol_type = other RNA
ctgaatagctgggactacaggtatgtaccaccacacccagctaattttttttgtagagatggggtttagccatgttgcccaggctggtcttgaactcctgggcttaagcaatccacccaccttggccccccaaagtgctgtgattacatgtgtgagccactgtgtccagtcgacagtagcctttttactgtgatgtcaataaaccaacatctgaagatgacaggaactggattcagagtctgtgtaaattttctcaatgagtgaccgagcatgtaaatttaactcaaatgaaattactacaataattgctttaaaaacatatttaggaaaatgaggtgaccctagatgagcttatttatatgtctcctctaacagaaatcacctcatggtaagagttgcttcttttggctcagttcacctgagaacaacttcatttggaacttttcttagccatttaacgtaacaggagactgactcaaagttggttctagtggatgaagcaaaatagacatgaccagcatggccaatcaatgagcttcattcaacggagcgtcctggccaagtgccacagccacgctggccagacacactgaccagttacgcatttcccaccagccaaatgccactgtttactaaaccatgatttcagtaggaaaaagagctctggaatcaaggccctcactgcagtacctgggtggggtgtccatggcctggcctgtagtaaaccctctgccttccactgtgttcacgttcgcagctctggcactggggcatctggcacttttttaaaagagatgtctctgcctctagatgaacaatctggaacttcagaatacagatcaaagaatgaagcagatctttcagtggcctcatcctgtggcacctgcccagccatttaactcccctgtcctcccaccctacataaagtgtttcccacaccagagtgtgcacaacatggtgactccaaatcccaaggaagttgagtttagctggaggttaaccccgtgctcagaaacccatctgttatctttccagcttcaggtttcagagcagtttataaatggcataatacaagggtaatgtgagtaaaatctgagagttttgttcattatcaagttatccacacagtgcccaattaagtaaggtgatctagtggagtaatacttctggcctgggagaaaaataaaaccagtcaaatcacacctttctctaaaatgtcccattaaaaaaatatggaataggccgggcgcggtggctcacgcctgtaatcccagcactctgggaggccaaggtgggcggatcacgaggtcaggagatcgagaccatcctggctaacacagtgaaaccccatctctactaaaaatacaaaaaaattagctgggcgcggtggcaggtgcctgtagtcccagctactcgggaggctgaggcaggagagtggcgtgaatccaggaggtggagtttgcagtgagctgagaatgtgccactacactccagcctgggcgacagagtgaaactccatctcaaaaaaaaaaaaaattatatgtatgtgtgtatgtatatatatgtatatatatatatatatgtatgtatgtatgtgtgtgtgtgtgtgtgtgtgtgtgtgtgtatatatggaataaagtttgagattccctgctttttcatgttaccttagcctcaattttaaacttacattgtttgttaaaattatcaaatggacaacctcattgctatggaacaaaaaagactgtgaggaaaaagaatcataacttggaaaaaaataagtgaaaaggcattgagagattgctaagatttgttaagttaaaacaataatatatctagaaaagactgtgaaaatatatatctcaaaagagaacaaggcatagtcagaaggctcagtaaaacaattactttaaaagctgactaataaaaagggtaagtgaaagaactcttccatccttgacccttcctcacttcctccctccgactccaccagtctggatgcactaaagcagaataacctaaaagccatgaaaaagtgctggtatttttcaggatctcttcaagacaccttccgtcttggtaacctgaattctctctctgatcaaggcagctgatggactttcaatgtatttggagatgccggttcaaaaacgtcatcatcatcttctgctccttcttctatcggtttcatcttggcagaggctcgctggtgtggggatgacacatgaagagaggacatgctggaggtaccccgaagaaactggtgcaagccgtcgtcactgtcactggagctggctatactgttcctcatttccaacatggagatctgtgtgcagaggctgagctgatgttccagctttttggcttttttatcatttaaggtgggatcattcaatgagtagagcttatttgtgatgtcttttccaataagatacctaaagatttcatacaagaaaggttctgattccagaaagtatgttaatctttctcttgaccagcataaaaatctgcagttatcatctgcaataatggtgacctggaatttttcacctttgtgcatctgagttgatctaaattcaggagaatctataaaggcacaggggtaaatgttatgcagaaaatgtcctcgataggagaccttcatttttcccttcaagagaatactcagacggtcatcaactgaggttttatcctctgcagcataagtttggccctttttcaaggtttggatcatgcaaaactgtccagttagtcttctgaacaaatctggaggcacacggagtggttcaaacaatcgccggtacatgccactgagttccttttcaatctttaccggtctcttcttgtataaaagatacgacagatgcaaaatgttgacacccaagaacacagagttccagatcattatatccaaggcacatcggtagagagtggcccagacgatataaagggtacatcctagagttaacattcccctaagaaatatcatatgaaggtgaagagtagttggaataaccaacccaactgcaaaacaaatatttgctacatgaaaaaccagatgatgtatctctctccagttttcacaagtggtcttattggaaggcacaggtatgatactttctaactcaggtgtaaaacctatggcagttgattctctcaatgggctggactctgtataattcattttgaaaattcccggctggtccctggcggggagcctgggcagcgccgaccaaagttcggagcggcagcttcggggcgcgggacgcggggcacacgggctcagctgctcgacgggagcccgacgcgcgctcctcggcgggtcggcgggtccggaagctccgctgcccgggccgggtccccaagcccgcagccgctttgact

SEQ ID NO: 10920 - RNA, 9660 nt, Homo sapiens
  source 1..9660: mol_type = other RNA
ctgaatagctgggactacaggtatgtgccaccatgcccagctaattctttttattttggtattttttgtagagatggggttttgccatgatgcctaggctggtcttgaactcctgggttcaagcagtcctcccacctcagcctctcaaagtgttgggattacagatgtgagccaccacacctggccttggactagtatttcttcatttgtcttttttaagtggggaggtgggagtggctaacttttttcattattacgtgtttatttttccagatgaagtttggtgtaattttatcatgttaagagattatttcgtttagcattgaattaatagatttagggacatctgtacagttctgcacttctgagctttttttttttttttttttttatccaaaagaaagctatgtctggttaggtaaatcatacacctgtatccagagttttgttttgtttttttttttaggtttttctttttaatgaaggtcttacaactattttccttttattaccactacgtacttctaaatattaatgtttttacaaaagcactgtaatggttttttttgtttttaaagaaataaattttcagttacttcttttggatgtcccagatacactaatcgtttgcaagtaacaataatatggcattctcatttccagccttcacatctcaggagagtattaaagggtggtattggagcacaccctcaggacatgtttgttttcaaatttagattctctgtggccattccagcctctatagagatctgaaaaaaacatttagtgccaccctctcattttatagttcaggacacaagcccagaaaggccacacaaggactatgtgtgtcgtaactgagagtaggctctgggtctcttgacccactgaacagtgctctttcactgtgagatgccagtactagggaagctcaccttcagatctctgctaggtcactccctggctgcaataacctagtgagactgcggaaatcatccagacaggttttaaaacatttttttctttgtttcaagtaatgtctgctgtatatgacagatcaccaaagaaaatactggcagtagtgtattccttcagatacttgacctagaaaatttcagtatgagagaggcaaattttaggtggttcacaaaaccttagcttgttggcaagtttagacaaaattatattttctaatttgcctgtgctttagaaatttggtgtgctcagtccatcagaggggcggactggggttttgcttttgccttaatcaatggcaagatactcttgcatgttggcgcttattgaacacctactgtatttcaggcactgcaccacagatatgcatacaaaaataagagagaccagtgtgggcaacaaagtgagaccccctctctgcacaaaattaaaaaaaaaattagctgggcatggtggtgcatgtctgtagtcccagctactcaagaggctgaggtgggaggatcactgaagtccaggaggtcgaggctgcagggagctgtgattgtgccgctgcactctagcctgggtgacagagcaagaccctgtctcaaaaataaaaataagaaagatggactctgtccttgataagcttgttctccatttagatgcatctatttgaaatttgattttctgtatttcctctaattttccaaataaaaaaattttttgactctgacttgggccaccttctgaaaacatttcagacacatcactaagttgttgcacatcttttttaatgcagggccagggagataatccaggagtttgagaccagcctgggcaacatggcgagaccctgtctctacaaaaaatactaaaattagctgagtgtggtgtgtgcctgtagtcccagctacttgggaaactgaggtgggattgcttgagcccgggaggcagaggctgccgtgagctgtgatggtgccgctgcactctagcctgggcaacagagtgagacactgtctcaaaacaaaccatgcaaagctgattagaaagggtaagtccctcaaggatagtgcccatcctttaaaaataactttctgcttgtactctactttggacctggtaagtttgctaggtacggcttagcatacatcttattgaaaagttttagtgtccaggtgcaaggcttacaattccctcctcatgctaaatcagcaaggctccgttcctgtttcagtttcagttttggaacatgctgtcctattttagcatgatgttgaaactaatagaatagacagtgacacaaaagcactgtgcagattttaacgtggccagttaggcctggctgtcctttgagaagaacctagttgatgttaatattaacataaagatagtaggggagttttttttttttttaaattataagaaggagtgcaggataaaaggctggaaccacattagccgaaggtaaaagcaaagactggtgtggtgttgaataaaaacaggggaccattcatactaatggctgtatttaagtcacccaaggcacatttgggtggtgaggagactgcttcgtggtggtgaggcatgggtgcagtgagttgttatgccaggaaaggagcacgattaagccagcggtctccattagaggctgcttggcatcctgggattgaagccaggggactgactcaagtctaatgtcttattctcagacagtattgatgctaaaaccttttgaatactgacggaggtaggaatttatcttgtgaagacctctagggatggaaaggtccacactgtctcctagaagctcttccacatgtccctaggcagagctattccatagtgtctccattgtgtttgcattagcactttgccctttccacctagatacctgtcatgtcaagaaaccatcaccttccttaacaaaagtaaaacccagaaactccactggggtttttgctgattttctttgctggctgccatcaagatagtccccagcacagttgaagggcatctaaagacaggcctgacagtttaagaaactgacattgaagattagagaatagcagaatattatagctattatgtaatattaaatccagatggctgttctacaagtttaatgtgcttagaattacctcacagagcttggatccatgaagtctgaggaggaacttaggagtctgtggtctgactgaggcagtcctgggaccactctttgagaagcgcagcgctgcagagatcatctgctttatgaggcacagtgggcttgggcacaaccccctctttcttcatcttacagcctggatattcacttacctgttgattgcaactctcagccattagagtcatctggggaagttggaaacaaacttggcccctctcccaaccaatgaaattgggatccatagtgggtagggcccttgcagtggtcacttttaaagctcccgtggttcaaaggtgcagccaggattgagaaacactgcgttagcatagactttgctccctataagatgcatctttgtttgctctaccaggcactcttaaggctcatcttgggtatttatacttcagggtaaatagattcagaaagggaaacttgataacaaattgagaggctaagggccttgatacaactctcagtttgtccaccttttgaccacttagttggtcttggtgtaggtctggggaagggtgtgaaggactgtggagttctggaataagggctgcttgcctctgaccgagagtccagaggttgcaattcagtgacctctgggctgcatctgaccagcaggtacattctgtttggcctgcagtgtggtcacaggtggcagtttttaaaaatatgaatgccagcctctaaaaatcagatatccataagagcattctcagatctgatgatatttgatggacgacttggtgctaagtcaatgaaaacttatgagtgtgggttcattaattctcatttagccaggttaccccattcataagagtgatgacggaaatggaatatgatttagcaacatttccttctgattctattagaaggcaatgggttttgatactcaaattttagtttcaccattttcaccttttgctccacatcaagcccttctaaggctgggctcgaataacagaatctggcttgggaaatagcagtcctgggtttagttttggttttgctgtgggagcctagggctcttcctggttctgagtgtcctcatttatgcaaaaacaagatcaaattatttccaaggttctacttactgggaatccaagacatgaatggcacaagaacagaatggagacgccttggctgatgtcagagtgtaagacggttaacaatgaaaccggcctggagaagtctgggaggcgtgagagggaagagctggaaccaagggcagaagctacagtgaaacatttaggtcctaaccgtccacactggccatagatggaagggtgatcttgggagagggagcgctccaccactggagacgtcacacggaggccaggcagccactaggagggcatgttgtgggcagcaaatggtggatgagtcccttctgacatgtagaggtaggggggaggaagcaaggaactccctcattctacttcctctccttcaaaggggagtatggctcactgtgatatgctctgcccacagaatgggatgtcagtgcttggttgtttttaaacactgtatttttaatttttcaaaaatacgacagtaaaggtcgtactatgcacagggggactgatgcctttcatgtgtcccccttgcatttctacctcaaaacaagactaaggcataaattactccactgggcgccaggcacgccccttgtccttggggcattatcactggtcataccacttgtcctgggggccggcagatgagatatttgccaccaaggctgcacaggctccgggagtccttgcacgtgctttattcagtgcattccagaggggacccctcaacagcgctggccaagcccttccctgtgcactggcgggcatgagggaaggatgggaggcagtgtgtgtgtgtgtgtgtgtgtgtgtgtgtgtgtgtgtgtgtgtgtgtgtgtgtgtgtgtagggagggggtgatacagggaggggaggctccctacccctacccctgctgcccagctgcagccaggccggtgcgtccatgtctaggggcaggctgcagcaagaagacgtgggaatgcacagccccagggattgtgtcatccacatgcttcccatgaggtacctgggaacaaaagtgacccgggagggttggcagctgagagcaaggggctgcagctggtgggggaatgtgtgagttgcggtcaatgtgaatgcacgtgggtgcagagcccggctacctctcatctcaggacagcgtccagtatcctggtcccacttgcctggccatcagtctccacatctcagagtctttcttcatccctggcttgcagctgtcaccatcaagcccttgctcttgggttcattcttcgggagccccaggggcctatctatggggaagggagtgggtgtgacttgggagccaatggaggggtgggatgggtgagagaaaagggcagaattcagatctgttttgtcttggatccttctggaactagaggcctggagtgtgcagattgggttcgtatttacagtcttcctccctgggtttctctggaggatggggatgattacgaattcctagcaccttagtagctggggcagcaaatgccctccacagagcctgagggaggccttggcatgggcctgggtgtgtgtaggggtgtccctttaaatccctaggggtctgtgttaaaggtgtcccagtctcccagtagggcagttccacttaaaaccagcttgagttccattctggagggagcaggcgccattgctcgggagatgaggtcaagtgcaaagccagctggcttcctctccgctccagctcggtggggccacaggcctgggtctcaacactacctggactggtgtcctggcccccatcaactcaaagtctcctctggagcctcactccagcactttgggggtggggtccagaccaggctccctcctgcgcctggcacttctaaagaagccgagcttccacagtgccaggaccagcagggccagcagtaggaggccccccagggtgctgcctacaatgatccagatggggacctgccagtcctcttgcttggagatctcaaacacgatctggcggctgggatcctcctcacggaagatgaaggggctgtggaactgcctctgcaaggctgcgttgaccatgattttcatggatttgtacttgagtgcttttagggacctcaaccacaggttccccagtagatggaaattgatttcctggttggggaccagccgtatattgcagttgatggagacgacatcagagttgctgtgattcagctgtggagcacgacgcaagtcttcctccactggggtgggccggtactcagtgctattgccccagatgttacaggacgtgttcgcctcgtccgtgaggaagtccctcagcttcagtaggcggttgccgctcctggtggcgatgggaatggtgatcttcatcatcatcccgtggatggggaacaagcccaagttctggatcctgaagatgcagctgaagggaggcccgataccatcgtatctctccagcgagctgttgggcttgacctcgtagtggctcaggctgctgctcctggtgaagaggacgtcagcctcgtatttgaggtggaagcgtaagggggccacgttgtcttccttggtgctgtcccgctcattactgtcactgcctgcagcgagctcgatctccaggtggtgtaggaagatggatttgctgaactcaaaatcaagacggaaagccaccttggccttggcccggaagaagggatagctgacgttgcagacttgcttctggagcctcctctcctcgttcacacactcaatgctaccgtctgagtcctccttctggatcaagctggcaaactgcaggtttgctgactgcgagatatttaggaccgtgctgtaggcgttctcgcccctgttctccagtgtggcctccaccgccactcgctggcgtgtgctctctatgatgaagactgtggtgtcgaaggacagcgtgtatgcggagcagtcctgcgcaggcttcctcagcaccctctggcagtactccatggccgtgggcaggtcactccgggcatccaacacaaggtcagggacacagtgctcatcctcattgcagccgttccagaagggcaccgagactctgagagtggtgggccagccgtcgtccagcatggggccatggtcagggtcctccagggaatactcgactgagaaggtcactggcttcacgtagtcagcagtgtccaggacatggaagttgatccgctcacagagctcctggccggaggagagcagtacggctctgttggtgaatcggtccccgccctcgtccaggtgggccctcggtgtataccgcctctcatccatggtggcgttgtatctgatgccaacagttgttgtttggaaatggggtgccaggaagatgggcgtgaagcagaggaaggcggccaggcaggtggcatccctgccactgcgcttgcagtctctgtggaagatgttgatcttggatggctcaaagtggaggctggcattgatctgaaccactgggcgggaccacagaatcacagcgttgccaagggctcccactgccaggtcgatgagcccatcctcattgaggtccaattgcccgtggatgctgcagccaaaatactggaggccggtagccagctctgaggctgtgattctctgcttaggtgtcttcaggatgctgcctcggaagccgtggaagatgtagatggctcctgcgtggttgtcctccaggggggctcccaccaccacgtcattgtaggaatcctggttgaggtctcgaactgaggcaatggaggacccaaatcgggcattctggtaactgtgtgaatcctttagcgttccgttataaacaaacaggttctgtctcagctcatagacgtacaccttgcctcgctcacggccctcgttgaagtacatgggtgcgcccaccagcaggacatcagtcacgccgtcgccgtcgatgtccaccgaggtgatttcactcccaaagtaagagcctatctgctggccccgcatagcctggtggatggtgaggctccggttgttgtgcatggtgaacaggatgaccttgcccgtgtggttgaaccggggggctccggccacgtacacccgcccctgcctggaggacacgaccgatgtgactgtgtaccccaggtatgcaccatggttcttgagctcctcggggaactctttcaggtaggactcgcggagaggaatgaccttcccggcactcgtctcctttagcacagctccattccagtcataggcaccgacggctcccagcagaaccccatcctccaccacgtgcgaggaaaagcccgtctgtgacatctccagcccaaaggaggtctcgttcttgttggtgccttccaggctgaagattctgtcccccagggcatcgacaatgtccttcaaggcagcctcatcagtgacattgaagaagtgcttgtcatcagggtcactggcgatgtatttgatttcatttagaaaagtttctggattgatccccctgcggttgtagtagcccaggacggccaccgcatatcttgttacgttgtctctttcgctttgctggatcaccttctccaggtctgggctgtcgtgggactccccatctgtgatgacaatcatcaccttcttggctcctttccttccacccttctggaaagcctctgagcgtgcaaattcaatgccaaatgccgtccgggtctctgttcctcctctctgctcaatgtggctggcagcttccaccacatcttttacagacctgtagtcgttgaggtgaaactcatgcaccacatcttcgccatactgcacaactccaacctggatctgccctgggccaatgtaaaactttttcaggatgttgatgaggaagtgctgaacctccacccaggggtagatgctgttggagccatccaggacaatgacgatgtccatgtaggtctggcacctttggagagctggggccacggtcttggagaacctgaagttggagttgactcttgaacacatccctgtggtgtagtaggagctcccacactcatgagaccagagggggctgcaggccaggaagctgttgtccttggggttggtggcgagactaaggccgaggcgcatgttgtctttccgctcggacacgttggacagggtgacccttcccaggttgagtttggtgcagttcccgtggatcactggacacttgtacacgtctcccgtcttctggtagccattggtttccagtggggcgcccacgaccagccacttattgccactgatgtcgtgctgctgcactgtgtagccaaagaaggcggtcctggagccagggatgacccggggcttcctggtgtccatgttgaaggtgtccgtgaaccctggccacaggctgagcgcccaggccaccaccaggcccctgggcaggtccatggcccgcggcacggcggctgggtccggtgtgcagcggcggcggggggcggcaagccagagcggcagcctcctcggcgcggcgcctgcagcctgcact

SEQ ID NO: 10921 - RNA, 1631 nt, Homo sapiens
  source 1..1631: mol_type = other RNA
ctgaatagctgggactacaggtatgtgccactgtgcctaacaggcattaatttatgttgaactttttcttttacttctacaatatagagtgtttaaaaacccttttctaaccatctgagagatgaacgatggttttattctttatatttaattgtttgtcctgtatggcatttattttgataagttgtgtggaaaaagtattcatcttcctcctttcctccctcctaccacccactctctctgtctctctctctgtgtttcttcctgatttcaaatagcttttctaacattttaaaacttgtctctcagcctgataccagaggttacttcttgagaacatgtttctccagtcatgattgtgtatacacacacacacacatgcacacacacacagaggagagcagtgttacagtactggagattgggggataaccaaagacaagactgagggggaaagtgtgtagtgatcatctctcagttcaagcctgaaaggaatctatacattttttaactactgaaagccccatttccctggggcccacttcctctgcaatgtatggtctttctgagggctgcctttacttcatggttcctcagacagtaaatgatggggttgaggagtggaacaatgacagtgtagagaacagataccactttgttggaattgtaggcatacatgagtttgggacgggcataggtgaaaagtgtcatggaatagaagagaattacgacggtcaggtgggaggcacaggtggagaatgccttttggcggccctgagcagaagggatcctgaggatggtggcaaggatagcagcgtaggatgccaccacaacacaaagaggaatagcaatgaccatgagggccaagaagaagtccaccatctcagcctgtgaggcatcctcacaggagacgttaaggagtggagagatatcacaaaagtagtgattgatctgaggcatgccacagtagtgaagttgtgctataaaaaccatcttaatcatggcagtcatgagtccacagaaccagcatcctccagccagtgtgccacagagctggttggtcatgatgactgggtagcgtagtggattacaaatggctacatagcggtcaaaggccatgatagcaagaaggatgtactcagtgcagacaaaggtcacaaaaaagtaaagttgagtcatgcagccattgaaggaaatactcttgtcatgactgaggaagtcaacaagcatcttggggctgatgactgtgacataccacatctccaggaaggagaggtggctcaagaagaagtacatgggcttatgcagctgcccatcactgtggatagctaagatgataagaagattctccagcagtgtcagcagataggttgccaggaaaatggagaaaaagagaagctggaaggctggtcgtgttggaaaccccagaagaatgaaacgtgttgtcactgtatgattatctacttccagaattatggtggtcatgactggcattttctcaggaatataacccttttcccacctagctttatcaaagatggccagcttgcgctgagaaaagagaagaaatcatgtagaccaagagaagaacaatgtacataagcctagagagtttctgggcaagtctggtt

SEQ ID NO: 10922 - RNA, 3057 nt, Homo sapiens
  source 1..3057: mol_type = other RNA
ctgaatagctgggactacaggtatgtgccactgtgcctaacaggcattaatttatgttgaactttttcttttacttctacaatatagagtgtttaaaaacccttttctaaccatctgagagatgaacgatggttttattctttatatttaattgtttgtcctgtatggcatttattttgataagttgtgtggaaaaagtattcatcttcctcctttcctccctcctaccacccactctctctgtctctctctctgtgtttcttcctgatttcaaatagcttttctaacattttaaaacttgtctctcagcctgataccagaggttacttcttgagaacatgtttctccagtcatgattgtgtatacacacacacacacatgcacacacacacagaggagagcagtgttacagtactggagattgggggataaccaaagacaagactgagggggaaagtgtgtagtgatcatctctcagttcaagcctgaaaggaatctatacattttttaactactgaaagccccatttccctggggcccacttcctctgcaatgtatggtctttctgagggctgcctttacttcatggttcctcagacagtaaatgatggggttgaggagtggaacaatgacagtgtagagaacagataccactttgttggaattgtaggcatacatgagtttgggacgggcataggtgaaaagtgtcatggaatagaagagaattacgacggtcaggtgggaggcacaggtggagaatgccttttggcggccctgagcagaagggatcctgaggatggtggcaaggatagcagcgtaggatgccaccacaacacaaagaggaatagcaatgaccatgagggccaagaagaagtccaccatctcagcctgtgaggcatcctcacaggagacgttaaggagtggagagatatcacaaaagtagtgattgatctgaggcatgccacagtagtgaagttgtgctataaaaaccatcttaatcatggcagtcatgagtccacagaaccagcatcctccagccagtgtgccacagagctggttggtcatgatgactgggtagcgtagtggattacaaatggctacatagcggtcaaaggccatgatagcaagaaggatgtactcagtgcagacaaaggtcacaaaaaagtaaagttgagtcatgcagccattgaaggaaatactcttgtcatgactgaggaagtcaacaagcatcttggggctgatgactgtgacataccacatctccaggaaggagaggtggctcaagaagaagtacatgggcttatgcagctgcccatcactgtggatagctaagatgataagaagattctccagcagtgtcagcagataggttgccaggaaaatggagaaaaagagaagctggaaggctggtcgtgttggaaaccccagaagaatgaaacgtgttgtcactgtatgattatctacttccagaattatggtggtcatgactggctgtgggcacagacaaagtcagttccttccatgacacaagcactagtctatggttatttgtattgatagagcccaccaccagcaaatttatcacaataggaggtttctgcttttttatcttactgcctcttgaattatgaagagaaccaaagcttttgagaaaagatggaatttagggagcttatattttaacttgttttcagattttctcaagagcagtaacttgtccaaggtcatacaaaatagagtttataactttctaaatcccagttctgtgctttaccaatatatcacttttgggcacataaatggtctccagaccaccctttcactacaggcaaaacatccccatctgctgaatatggagaagagaaagaaggcccaactacccattctctaggggcaatttgggtgactctggagtggttgcatgaccccacttatctgtaaaatggagagaacgttcttgcttgtgtctaacaatgtgcttaagcttgaatgaagcaatagttgagcatacccacaggattaacagcaaaatcaggtttgatgcaattattcaccagcttttcagagaacaaaattgaatggataacatgaagggtaatagtttcttcaatacaatccattgtataaagtgcttgcttaggagtttgacaaaagtgcattcaaatccaacttttgtctttgtatagctaagtgagagtaccacataatcttttagaatattagttactttatttctaaaatggggataatacaatggggttcacattttgtgaacatcaaatgggatttagagtttaaattcagttcctatgatatttgctgtgacctttccaggctactttacttaccccacatacatagctcctcctccttttaaaaaaacacacactccaccccacacaaagtttcccccaccccaacttcaacccctgccaaaaacagcaaaaaactggtgcaaacagcagccattgttaatgaaaaaagggagaggaccgtgggacttttccaagggtaataaatttaaaaactgtaatctgttgggagtaatatcagagaaaacaagcaagaattctattagtgactcttctgcatttctgttcattaatttagcaaaatgtgtgacctctttttgtgttaggctgataatcattcccaaacccattgatactaaacaccttcccatttcaagtcttgctctgtgtcctattgcttcaattctcttttctgctcttctccagagccacagtcactcttgatccccatttctcaacagctctattttatggcataaatatgtaggacaactaggggatggtttttttttttttttaaggaatgatcatgaggttgcagagccagaaaactactgcccatactatccatttcctcttcccacttagatttcagctttagattccattttctcaggaatataacccttttcccacctagctttatcaaagatggccagcttgcgctgagaaaagagaagaaatcatgtagaccaagagaagaacaatgtacataagcctagagagtttctgggcaagtctggtt

SEQ ID NO: 10923 - RNA, 2893 nt, Homo sapiens
  source 1..2893: mol_type = other RNA
ctgaatagctgggactacaggtatgtgtcactacaactgactaatttttaatttttttatagagacacaggatctcactatattacccaggctggtcttgaactcctgagctcaagcggcccacccacctcagcctccctaagtgttgggattacaggcatgagccacggtgcctggctatcacgcaattcttaagtgcttattccagtagcagaagagattagaaaggctggctttttccaacagtgggagcttgaatctggaaagtcttaaagttgttgtaatttcacactactaagaagcactttgctcatgcaactgaaaaaaaaattaagtgcctacctgggtgattccagggcacttataagcaactaagactaattagaagtcctcatagcctctaatgaaaagataggaagtaattcgctctatgatacaaaaattcctggatgtttggaattgttttacatcattgggcacaggattccttactgggagcttttgctttcccagggccaaagtccctgttctatgtcacacattgtggagggcaggggacaaatggatacagagcttggtatccactgatatggctcccacaaagacatttgggaggatgagtaaggaaagagagaggcaaaatctcagtaccagttgtaactggaaaatgtcatttacatggaatgagaacttacatggggcgagctgagaagcactttcagttgaagcaaatagaaaaattaaggcactttcctttacttttagttatttttaaacacgtatctttatgctcagatctttcttttataactgggttataactggggagaataaaaggatccgggcatgagagaaagtgaaatcaagggaggaagagggcatgcaatgggggaagggaggagcaggaatgtccactttactgaatacaaaatactgtaaaagatggatcctgccatattcttcccccaatcaacttggatgaaaaacagaaatactacattcttaaacacagttcatttttagtttgtcgtggcaatacatggaaaaaaatcaggccactactaagcatctatagagtgtatctttggcaaaaatgtggacctgcaacaattcagatggttttctttcaattaggttcaaaaatcatggctctgtaaatttccaaaacttttaaagtcttctcatgtcttcttataatcgggcattcagaggtacgtgttggttctaatagctttggtagaaacatgctgaaaatagaaatgaatataaaatgccttgtctttaggctaatttggtatggattagtaaggcctgagtgaactggaaattagtacatttcttgaaataatacaaatgaatgtgagacacatgggtagaacagcagattcagaaaaaaaggttagtattgtagtcccaagttttataaaagacatcaagtaaggccagcaatagaggaatcaagtttctttttcgggttccctggggtgatttcctatcagcttcacgttcatgagctggggatttgtaaaatgtgagatggcctttgactttgtttttgatgcgatcagcagcggcactgtctgcaatccaggcccagcattctcagacagcgtgcagtacggatgcttctggctggcagggaggtcgtggcagtgggctgactagtgtgctgtgttgggagggctcagagggtgatggggcaagcctccgtgcaaagggagttcctttctggtcgtgccctcctttttggctggagcttggccacagagattggctgccattctcatccctggatggggtggaggcaggtcccagacaacctcagataattgaacagcagctgtgaccctcagaacagcgtttcttctttttcttggggtggaaaatggtgaggattgcttcatcaaaaaccgctttgagacctttctgagtcagagctgaacattccaagtagcactgtgctccgatcgcttttgcgagcttcacaccatgctcgtaagtgagaggtttctctttcatatacagcaaacgggccaaggtttttgggtcatcacggagatcaatctgggtccctatgaggacataaggcacgtgaggcatgcagtccttgagctcggggacccattcctcctggacattgtggtaagaggcagggtttacgacagagaagcagatcaaaaacacatccgtgttggggtaggagagtggcctcagctggttgtagtcctcctgtcccgcggtgtcatacagtccgagcaagtgttgcttgcctcccacagtcacagtaactgcatagtggtcaaacacagtgggcacgtattcctctgggaaggcgtcgttggcgtagctcatcagcaggcaggttttccccacggcaccgtcccccaccaccacacacttcaacatcttcttctcgtcgttgcccctgcagccgcagctgctgtcagttccctctttgcagttcattcttgcggctccagctgctggggactcctgctgctattgcttctcctgctttttccaaagcacatgaagcggcagaaagccagtgccaggcttgagtttactctgtctgactttgggtaccttggatcatacagacatgtccgaggctgggatatgtcctgttgcttaccatgctggtaaagaaaggtaacacacacttgagggagttatgaaaagggtctgcccctttccgctctcagtgtgagttaagaaaccctcattttcacagaattcgaggggcttcctaacagcctagaaatttcagcagcctgagggttttactctgctctccctgtctctagcctggcaaaagatacggtggaattttgctaaatctttctcattttccaagtcacatctaacatggaggaaagctgggctttttaat

SEQ ID NO: 10924 - RNA, 2759 nt, Homo sapiens
  source 1..2759: mol_type = other RNA
ctgaatagctgggactacaggtatgtgtcactacaactgactaatttttaatttttttatagagacacaggatctcactatattacccaggctggtcttgaactcctgagctcaagcggcccacccacctcagcctccctaagtgttgggattacaggcatgagccacggtgcctggctatcacgcaattcttaagtgcttattccagtagcagaagagattagaaaggctggctttttccaacagtgggagcttgaatctggaaagtcttaaagttgttgtaatttcacactactaagaagcactttgctcatgcaactgaaaaaaaaattaagtgcctacctgggtgattccagggcacttataagcaactaagactaattagaagtcctcatagcctctaatgaaaagataggaagtaattcgctctatgatacaaaaattcctggatgtttggaattgttttacatcattgggcacaggattccttactgggagcttttgctttcccagggccaaagtccctgttctatgtcacacattgtggagggcaggggacaaatggatacagagcttggtatccactgatatggctcccacaaagacatttgggaggatgagtaaggaaagagagaggcaaaatctcagtaccagttgtaactggaaaatgtcatttacatggaatgagaacttacatggggcgagctgagaagcactttcagttgaagcaaatagaaaaattaaggcactttcctttacttttagttatttttaaacacgtatctttatgctcagatctttcttttataactgggttataactggggagaataaaaggatccgggcatgagagaaagtgaaatcaagggaggaagagggcatgcaatgggggaagggaggagcaggaatgtccactttactgaatacaaaatactgtaaaagatggatcctgccatattcttcccccaatcaacttggatgaaaaacagaaatactacattcttaaacacagttcatttttagtttgtcgtggcaatacatggaaaaaaatcaggccactactaagcatctatagagtgtatctttggcaaaaatgtggacctgcaacaattcagatggttttctttcaattaggttcaaaaatcatggctctgtaaatttccaaaacttttaaagtcttctcatgtcttcttataatcgggcattcagaggtacgtgttggttctaatagctttggtagaaacatgctgaaaatagaaatgaatataaaatgccttgtctttaggctaatttggtatggattagtaaggcctgagtgaactggaaattagtacatttcttgaaataatacaaatgaatgtgagacacatgggtagaacagcagattcagaaaaaaaggttagtattgtagtcccaagttttataaaagacatcaagtaaggccagcaatagaggaatcaagtttctttttcgggttccctggggtgatttcctatcagcttcacgttcatgagctggggatttgtaaaatgtgagatggcctttgactttgtttttgatgcgatcagcagcggcactgtctgcaatccaggcccagcattctcagacagcgtgcagtacggatgcttctggctggcagggaggtcgtggcagtgggctgactagtgtgctgtgttgggagggctcagagggtgatggggcaagcctccgtgcaaagggagttcctttctggtcgtgccctcctttttggctggagcttggccacagagattggctgccattctcatccctggatggggtggaggcaggtcccagacaacctcagataattgaacagcagctgtgaccctcagaacagcgtttcttctttttcttggggtggaaaatggtgaggattgcttcatcaaaaaccgctttgagacctttctgagtcagagctgaacattccaagtagcactgtgctccgatcgcttttgcgagcttcacaccatgctcgtaagtgagaggtttctctttcatatacagcaaacgggccaaggtttttgggtcatcacggagatcaatctgtcccgcggtgtcatacagtccgagcaagtgttgcttgcctcccacagtcacagtaactgcatagtggtcaaacacagtgggcacgtattcctctgggaaggcgtcgttggcgtagctcatcagcaggcaggttttccccacggcaccgtcccccaccaccacacacttcaacatcttcttctcgtcgttgcccctgcagccgcagctgctgtcagttccctctttgcagttcattcttgcggctccagctgctggggactcctgctgctattgcttctcctgctttttccaaagcacatgaagcggcagaaagccagtgccaggcttgagtttactctgtctgactttgggtaccttggatcatacagacatgtccgaggctgggatatgtcctgttgcttaccatgctggtaaagaaaggtaacacacacttgagggagttatgaaaagggtctgcccctttccgctctcagtgtgagttaagaaaccctcattttcacagaattcgaggggcttcctaacagcctagaaatttcagcagcctgagggttttactctgctctccctgtctctagcctggcaaaagatacggtggaattttgctaaatctttctcattttccaagtcacatctaacatggaggaaagctgggctttttaatggagtttttttccctttgcttcctccagctt

SEQ ID NO: 10925 - RNA, 3054 nt, Homo sapiens
  source 1..3054: mol_type = other RNA
ctgaatagctgggactacaggtatgtgtcactacaactgactaatttttaatttttttatagagacacaggatctcactatattacccaggctggtcttgaactcctgagctcaagcggcccacccacctcagcctccctaagtgttgggattacaggcatgagccacggtgcctggctatcacgcaattcttaagtgcttattccagtagcagaagagattagaaaggctggctttttccaacagtgggagcttgaatctggaaagtcttaaagttgttgtaatttcacactactaagaagcactttgctcatgcaactgaaaaaaaaattaagtgcctacctgggtgattccagggcacttataagcaactaagactaattagaagtcctcatagcctctaatgaaaagataggaagtaattcgctctatgatacaaaaattcctggatgtttggaattgttttacatcattgggcacaggattccttactgggagcttttgctttcccagggccaaagtccctgttctatgtcacacattgtggagggcaggggacaaatggatacagagcttggtatccactgatatggctcccacaaagacatttgggaggatgagtaaggaaagagagaggcaaaatctcagtaccagttgtaactggaaaatgtcatttacatggaatgagaacttacatggggcgagctgagaagcactttcagttgaagcaaatagaaaaattaaggcactttcctttacttttagttatttttaaacacgtatctttatgctcagatctttcttttataactgggttataactggggagaataaaaggatccgggcatgagagaaagtgaaatcaagggaggaagagggcatgcaatgggggaagggaggagcaggaatgtccactttactgaatacaaaatactgtaaaagatggatcctgccatattcttcccccaatcaacttggatgaaaaacagaaatactacattcttaaacacagttcatttttagtttgtcgtggcaatacatggaaaaaaatcaggccactactaagcatctatagagtgtatctttggcaaaaatgtggacctgcaacaattcagatggttttctttcaattaggttcaaaaatcatggctctgtaaatttccaaaacttttaaagtcttctcatgtcttcttataatcgggcattcagaggtacgtgttggttctaatagctttggtagaaacatgctgaaaatagaaatgaatataaaatgccttgtctttaggctaatttggtatggattagtaaggcctgagtgaactggaaattagtacatttcttgaaataatacaaatgaatgtgagacacatgggtagaacagcagattcagaaaaaaaggttagtattgtagtcccaagttttataaaagacatcaagtaaggccagcaatagaggaatcaagtttctttttcgggttccctggggtgatttcctatcagcttcacgttcatgagctggggatttgtaaaatgtgagatggcctttgactttgtttttgatgcgatcagcagcggcactgtctgcaatccaggcccagcattctcagacagcgtgcagtacggatgcttctggctggcagggaggtcgtggcagtgggctgactagtgtgctgtgttgggagggctcagagggtgatggggcaagcctccgtgcaaagggagttcctttctggtcgtgccctcctttttggctggagcttggccacagagattggctgccattctcatccctggatggggtggaggcaggtcccagacaacctcagataattgaacagcagctgtgaccctcagaacagcgtttcttctttttcttggggtggaaaatggtgaggattgcttcatcaaaaaccgctttgagacctttctgagtcagagctgaacattccaagtagcactgtgctccgatctggagtcctgcaggaggggcagggcactccccatcctcctgcccccagtgtgcagctgacagcatgtcaggctttgcctttcgatggagcgggaggagcccaagcttgtctcttccaattcagacatttcgcttttgcgagcttcacaccatgctcgtaagtgagaggtttctctttcatatacagcaaacgggccaaggtttttgggtcatcacggagatcaatctgggtccctatgaggacataaggcacgtgaggcatgcagtccttgagctcggggacccattcctcctggacattgtggtaagaggcagggtttacgacagagaagcagatcaaaaacacatccgtgttggggtaggagagtggcctcagctggttgtagtcctcctgtcccgcggtgtcatacagtccgagcaagtgttgcttgcctcccacagtcacagtaactgcatagtggtcaaacacagtgggcacgtattcctctgggaaggcgtcgttggcgtagctcatcagcaggcaggttttccccacggcaccgtcccccaccaccacacacttcaacatcttcttctcgtcgttgcccctgcagccgcagctgctgtcagttccctctttgcagttcattcttgcggctccagctgctggggactcctgctgctattgcttctcctgctttttccaaagcacatgaagcggcagaaagccagtgccaggcttgagtttactctgtctgactttgggtaccttggatcatacagacatgtccgaggctgggatatgtcctgttgcttaccatgctggtaaagaaaggtaacacacacttgagggagttatgaaaagggtctgcccctttccgctctcagtgtgagttaagaaaccctcattttcacagaattcgaggggcttcctaacagcctagaaatttcagcagcctgagggttttactctgctctccctgtctctagcctggcaaaagatacggtggaattttgctaaatctttctcattttccaagtcacatctaacatggaggaaagctgggctttttaatggagtttttttccctttgcttcctccagctt

SEQ ID NO: 10926 - RNA, 3044 nt, Homo sapiens
  source 1..3044: mol_type = other RNA
ctgaatagctgggactacaggtatgtgtcactacaactgactaatttttaatttttttatagagacacaggatctcactatattacccaggctggtcttgaactcctgagctcaagcggcccacccacctcagcctccctaagtgttgggattacaggcatgagccacggtgcctggctatcacgcaattcttaagtgcttattccagtagcagaagagattagaaaggctggctttttccaacagtgggagcttgaatctggaaagtcttaaagttgttgtaatttcacactactaagaagcactttgctcatgcaactgaaaaaaaaattaagtgcctacctgggtgattccagggcacttataagcaactaagactaattagaagtcctcatagcctctaatgaaaagataggaagtaattcgctctatgatacaaaaattcctggatgtttggaattgttttacatcattgggcacaggattccttactgggagcttttgctttcccagggccaaagtccctgttctatgtcacacattgtggagggcaggggacaaatggatacagagcttggtatccactgatatggctcccacaaagacatttgggaggatgagtaaggaaagagagaggcaaaatctcagtaccagttgtaactggaaaatgtcatttacatggaatgagaacttacatggggcgagctgagaagcactttcagttgaagcaaatagaaaaattaaggcactttcctttacttttagttatttttaaacacgtatctttatgctcagatctttcttttataactgggttataactggggagaataaaaggatccgggcatgagagaaagtgaaatcaagggaggaagagggcatgcaatgggggaagggaggagcaggaatgtccactttactgaatacaaaatactgtaaaagatggatcctgccatattcttcccccaatcaacttggatgaaaaacagaaatactacattcttaaacacagttcatttttagtttgtcgtggcaatacatggaaaaaaatcaggccactactaagcatctatagagtgtatctttggcaaaaatgtggacctgcaacaattcagatggttttctttcaattaggttcaaaaatcatggctctgtaaatttccaaaacttttaaagtcttctcatgtcttcttataatcgggcattcagaggtacgtgttggttctaatagctttggtagaaacatgctgaaaatagaaatgaatataaaatgccttgtctttaggctaatttggtatggattagtaaggcctgagtgaactggaaattagtacatttcttgaaataatacaaatgaatgtgagacacatgggtagaacagcagattcagaaaaaaaggttagtattgtagtcccaagttttataaaagacatcaagtaaggccagcaatagaggaatcaagtttctttttcgggttccctggggtgatttcctatcagcttcacgttcatgagctggggatttgtaaaatgtgagatggcctttgactttgtttttgatgcgatcagcagcggcactgtctgcaatccaggcccagcattctcagacagcgtgcagtacggatgcttctggctggcagggaggtcgtggcagtgggctgactagtgtgctgtgttgggagggctcagagggtgatggggcaagcctccgtgcaaagggagttcctttctggtcgtgccctcctttttggctggagcttggccacagagattggctgccattctcatccctggatggggtggaggcaggtcccagacaacctcagataattgaacagcagctgtgaccctcagaacagcgtttcttctttttcttggggtggaaaatggtgaggattgcttcatcaaaaaccgctttgagacctttctgagtcagagctgaacattccaagtagcactgtgctccgatttaggatcctaaggactccatggacgtctggcgctagttagtattgacattactgtgcatagaagtaggaagagttcagtatctcgatcaggtgttgtgagaggttctcatgcaggataccgcttttgcgagcttcacaccatgctcgtaagtgagaggtttctctttcatatacagcaaacgggccaaggtttttgggtcatcacggagatcaatctgggtccctatgaggacataaggcacgtgaggcatgcagtccttgagctcggggacccattcctcctggacattgtggtaagaggcagggtttacgacagagaagcagatcaaaaacacatccgtgttggggtaggagagtggcctcagctggttgtagtcctcctgtcccgcggtgtcatacagtccgagcaagtgttgcttgcctcccacagtcacagtaactgcatagtggtcaaacacagtgggcacgtattcctctgggaaggcgtcgttggcgtagctcatcagcaggcaggttttccccacggcaccgtcccccaccaccacacacttcaacatcttcttctcgtcgttgcccctgcagccgcagctgctgtcagttccctctttgcagttcattcttgcggctccagctgctggggactcctgctgctattgcttctcctgctttttccaaagcacatgaagcggcagaaagccagtgccaggcttgagtttactctgtctgactttgggtaccttggatcatacagacatgtccgaggctgggatatgtcctgttgcttaccatgctggtaaagaaaggtaacacacacttgagggagttatgaaaagggtctgcccctttccgctctcagtgtgagttaagaaaccctcattttcacagaattcgaggggcttcctaacagcctagaaatttcagcagcctgagggttttactctgctctccctgtctctagcctggcaaaagatacggtggaattttgctaaatctttctcattttccaagtcacatctaacatggaggaaagctgggctttttaatggagtttttttccctttgcttcctccagctt

SEQ ID NO: 10927 - RNA, 3549 nt, Homo sapiens
  source 1..3549: mol_type = other RNA
ctgaatagctgggactacaggtccacacaaccacaccaggctaatttttgtgtttttgtagagacaaggtttcaccatgtttcccaggctggtctcgaactcttggactcaagcgatccacccaccttggcctcccaaagtgctgggattacaagcatgaggcactgcacatggtcattgtacattttcttaatgctgctgtaacaaattaccacaaacttgagggctgaaaataacacaattctagatgtcagaagtctaaaatgcatctcattgagttaaaatcaccatgttggcagggctgcatttctggagattctagggaagaatccgttttcttgcctttttcagcttctagaggctactcacatttcttggctcatggcccccttcttctatcttcaaagccatcaactgctggtagtctttccctcattgtatcagtctgacactgaatctcctgtctgccttttccatttataaggaccctgtgattacattgggcccacccatacaaaccaggagaatctcccatctcaaggtcagctgattagtaaccttaattccctcttgccatgtgatatagtatagttataagttttggagattacagtgtagacatctttatggggcattattctgtttatcattgatgtctattcacattaatgcaggtaagaatatgtataggtattataaaattgataatttccatattcttcctctttcccacatttaaatactgaatactaattttccttcttttgaagcttgggcccattactacattagcactattactggtgactttaggttcatctgggcacagtgagtgcaataggaggagggatgtagagtacccatcatgccatgcactatgaatttgcggatacaggctaatcaaaaatttttgccttgggcttttttttttgagagcaggagagatttggtatcaatgtattaaaaaagcacttggattatctgtgaattctatatgaataatatagaatatattaacatatattaatatgaatgtaatatatataattatatatagaatatatataattctatagcatctgtgaatgctatagctgggttcaccctgccccttagaaacaaagaacccagaatcaaatttctaggtctcaacttcaagtgcctctcttagataataaagtgttaagtataatatgttctcagttatttcaaatgctgccagtgctttttggcttcagctaatctgtggcttgacttggttaagctactcaattaagagtaaatatccacccttacctcagtccttcaaaccttaattctttcataatgggataaaaacactcaatgataaagtttaacccaaaggtagacaattagaaaagcttatcagctgtgggtaaaagcacattgttttcccttttcccttcccttcccttcccttcccttaccttcccttcccttcccttccctcccctcccccctttccttcccttcccttttttctttcttttcttttttcttttcttttttttttgagacagagtctcgctctgtcacccaggctggattgcagtggtgtgatcttggctcactgcaaactccacctcccgggttccagcaattctcctgcctacctcctgagtagcacggattataggtgcgtgccactatgtctggctaatttttgtatttttagtagagacggggcttcaccatgttgatcaggctggtctccaactcctgatctcgtgatctgcccacctcggcctctcaacgtgttgggattacaggcatgagccaccatgcccagcatgttttctagcaagataacaaagaagggtgcatttggattcttgaatcttattccaagatcaactgagaatttagccataagtattttggaaagttattccacctccttcaaattgggttctctaccttatatattacataacaaatgaacacactttgatacttttcccaacaaagcctttggatagaaaccaagaagcttggtttgctattttcatgcttatggcatttgctcacctaacttttagttatgacctcaaaagaaaaggccctcctctcttcctcacactactttgctcattatatgtgaaattcaactgtccctttgaggccaactactaatttttcctttctgcttcccaagaaaattagagaaatttcagaattcaaatatgacaacttttacaagtcataggccaaccatcaagttgtcatctgtgatatggaaaggggaaggggatggatctaggttcatcaagccatggatttggcactgcttgacacaataagccttccagatgtctttagtgaattcataattaaaatagtcaaaaggatcaatacctttgaagaaacaatccaagctccaaggggcagaagtaggctgagtagtcactttaaattcaatcaatacatttaacaaatattcattgaatacatattaaatggtagtgttaggcactggctaataaaccaacagacattgtaccttatcaaatggaacttatgatctattgagggagacaggcaataaccaaaaaaaaaaaaaaacatataattatacattgtgataagaaaattaaagggaaagaaataggatgcaatgactaataatgaaaaacagcatatttactttagaaagagtgattagagaagaaatctgtgaaaaggtagtatttaaagccagatgtgaagggtaaaaagaagccagccagccgggcacggtggctcacacctgtaatcccagcactttgggaggccgagatgggcggatcatgaggtcaggagatcgagaccatcctggctaactaacacagtgaaaccccgtctctactaaaaatataaaaaattagccaagcgtggtggcgtgcacctgtagttccagctattcgggaggctgaggcaggagaatggtgtgaacccaggaggtggagcttgcagtgagcagagatcgtgccactgcactccagcccgggccacagcgagaccccgtctcaaaaaataaataaataaataaataaataaataaataaataaataaaagaagccagacattgaagccatccaagtttgcactttccatgtaatgtaagtaaagaaccaattgaggtagatagaggtcaggaaactgcagctaatgggccaaatctgacatgctgcatccttttttatagcctccaagctaagaatgatcttttacatttttattgatttttttttcgagttggagtcttgttctgttgcccaggatggagtgcactggcgcgatctcggctcactgcaacctctacctcctgggttcaagtgattctcctgccacagcctgctgagtagctgggattacagtgtgcaccatcatgctcagctaatttttgtatttttagtagagacagggtttcaccatgttggccacgctggtcttgaattcctgatctcgtgatccacccacctcagcctcccaaagtgctgggattacaggtgtgagccaccacacccagctgatcttttacattttta

SEQ ID NO: 10928 - RNA, 9445 nt, Homo sapiens
  source 1..9445: mol_type = other RNA
ctgaatagctgggactacaggtgaccaccacaatgcctggctaattttttgtatttttagcagagagggggtttcaccgtgatgaaaccaggatggtctccatctcctgacctcgtgatccccccaccttggcctcccaaagtgctgggattacaggcaagagccaccgcgcccaccagttctaagttccgatacatgtacttgctacttaagaaaaacatgccgaatttaaagcaaatagtactgtaataaaaaaatctgattttcctgaaaatggtttaattttatgatgtaaatgcaaatcttagaagtaaaaacttttttcaaagaagacttttatcagactcaattagcagttaaatgggtagagagaggatgtcagtgtacgagaagccatatggagttttgggtggccaggagcaggaagtcaggcaggtttggcttcagttgtactacctagagatattttggaagaagctagagtgaactgtgtacatatatgagtttagatttcataagacacttagctttactggagttcactgcagaaaatgagggaaagaaaaatgttctcgatgtatacaaatgccacagacagttgtttttacacctactttatttgatagcttctaatggctgaaggagatttcaatatcaagtagttgtttgtcacaaatgtgcctaaaaataactttaaagatctttgtagggaagcagaaactcttaagtccagatgttttctcaggataactaaacctggtaaaatcacctatatagaagtaaataatattttatggccacatctgcaaaatgaaatatgatcatcttcattgtcgatataaaaacaaatgaaagttatgggtaatttttgataaaatgaattatacaaagcatcatttatatttttatatttggctttgggacataaggcaatatggagaacttatgtgacactgacacaaacacacacacacacacacacacacaaactcaagtactcctctctgcctcatccttattcctttctgagatcagcccataatatcagtaatcctctgctgaactaaaataatatttttgctccaaaagtctgctagggaaaacatctattaatatatgtttttaaatcaaatatttccagaaatgcttacaagtccctttaaatctagcaatgatagcataataaagggcatattctagggaagaaaatgcccacctaaagtagaaatttaccagttaaaaatcacaaaacatcaaaaactattttcaaggattatttccatttacctaataggtttttccatttaaaagttataaaatatttaaaaagagaaaacagaacattcaaataaccttagtttttcagttttacaatcaaggagttggactagatgctattttttttttctcagctctaactataattttagtcaacataagaagacgttaaaatgtgtcccactggttcattcaactgttaatagaaaaaagtggcttaaaattgtgaagtctgaaagtatagccattctaatttacagataacaaaggcaagtcctaggaagaaaagtgaccacccaagggcatccatccattcagagatcaagcaatgtcactgttttcaaatctgcctgatcatcaatattttgctttgttttgttttgttttattaatggttctggagtcccagtccctacccctggaaattttgctttagtaatatggggtgagatcagaaatttcattttttaaagagatcctcaatattctaaggaaccacagatcataccagactacttgggatacactggtggagaggaacagataggttgcacagtccttgggcaggctctccattgtcacacaacagcattttcctaacaggtccgtcattttatgacccagggttcctctttcctggtgttttctcccctctagctggaaagcatattatgagagtgatattacttggtgtctagtttacttttctttgatagcttcctgtggaaaaggatcttcctgaaggaaataagaattaaaagagtagatgtatagaccttagttaccatccaatacaaatcactctagacctttaattccacttaactaccgaaactgtccttacagtaaagtatgaatctagacatcaccatgctacagtcttgagcctttcaaggaagtctgcaatttgaaaattattttctttacctcaggtcatggggtacaatgaagtgaatttctctaaatggttcaaatacatcataaggagatggctcttggaatacatttggcataagaatttcttagtaaaagaaaagcttaaatagagttaatatctaataacataacataattggttttatatagtgacagtagagagcaaagttccttctaaaatcttccatttagaattccaagcccctcgacattcatatttctgtcagttttcaatatagattttatgtgttcactgtatgcaaactgtagccaaaatacacatttctattcctgatgctactgtggatgtcaaggtttagtttaagccttttttcggtagcaaactgtgagaagtataatttcagctttcaaagaaatattattcctgatcttccttgttagtaaaaaagtaacttagtttgttatctattaattttaaggaaaagattagaaaaaggaaaaaaataataaatgacttacctctaagtatgtatgactccatgttaaagcagctaaactaaaagcttaccacaacttaaagaaaaactaaaattcaacatcattcagtttctttttgcatcccatttaggaaatgtttgttgctgaggctgacaaaataaattcatcatttaatcatgtcatttataatgcagtctcatgatactgtctctgaggatcaaatattcagttaaagccatactagactaccaaataatatataaaacatttatgaacattttatgcttgctttacaaggctgatctattaaacttgtgacatttttatttaaaaagaataaacaagaatatcaatggtattattttatccttatatgggttaagaaattatttatgagttgtctttagaaatctaccaatgttagatgtgtgcataattcttctttttcattgtagctgggggccaaggaagtggtcaattaatatttgtactgcaaatgccttaagtggatacctattaaaaggtatacaaaatataaacagtactgcatattttcaaaacttttaaataaacacaaagaatatataggtatacatgttataatttcaaagtcaacactagcacataagtttttcatatctaaatacatactaggatacttcctatttcaacacatgcacctacaaacacatggccatgcacataaccttactttctgccacttgcaacaaagaatatacaatattgtacattgtttcaacttatattgtattggaaaactaatgaggatggcattaaaaaattctgatctaagaaatcaaaatgcaggaagataattattccttagattaaaaacactgaagactgatggaaagttaagattcaaattgcttgtcggaagagaacaggtccgcctgtaaacactcagaatgctctgtttgacaagtgggactagaacttctgtaatatagcaatccaggccaaagacttaaaccatcaatgcttcggatcgcagagaaatggtatagttgtgggtagttctccgcaaggcagggggtgcagatggagatctggatgcccatctggaggggagacgacgatttgctggtctagcaggtcgggaaaatccttttccatgtgaggcgttcactgacatggattcctctgttatctttttcggatctattccttgcttcacttcctgtcccccccacacagctgtcttttgctgaaactgttgttccatttggagcatttctaaatgctgacttaatgtggcaccaccactgacatcagaattacatttggtccaattatcctggaagcacttagaattttgcaatgcagactctgttgctgtctcataggttttcagcagcttttccacaacaccataatttgacctgggatcagctgacctcggacggccagacaaattactcggtctccagtcatgctcgtggagcatatttcgataactgcgaggacttaggtgtccctgcatttgtcttactaggcctgttgtggatttcttggtgggattatcaggcacattttccatgggcacaggcatgtgggcattggttttccaaataccggacacatcgttactttgtgatatgctacctgtgtgagtagatgaggtatcacagggcttgagatcctccgatgattttgagcagctgtgattttgctgtattgcctgacaatttctatctgttctaaatacagttctgttaaattcatcagtctttgctgccagcttctcattccttgtagtcctttcaaagccacaactgaaatttctaagtgggctactgctctctgctactgaggagctacagtcattacttacatgaagatcaggatgagatttagcagggtgatctgggatcaccatttcatattttggattactgggggtagagcaggttttctgaaaccacgaagtagaggggctcctttttgcacctatcccaatgtcacatgaccacatgctaagtccaacatcttcattacttggaggcttgctatctattttgacttctggtaccaaagaggaaaagatgataccatctttcgaagttttcccttcatttggatacaacatagacatctcttgttgtctcaaagggaagtgagggttgtaattccttttacttcgaccctcatggggcacccagctgttgtggtctaacctttccttccatctttcataggcttgttcagaatccgagctgggaaaatttcgagaggtgcttcttggaggaggaactggtggagtttcatttctttttaaatcgattgtatcaattccacattttttcgtagaattgctctggagcacattggtacagctcagattcttcctgtttttctgtttttctttttctaaactgattggaagaatgcactggtcattgttgatcatggggtccccatgaggtatattagttacatttggcatttcctggagaaaagaatctgacttcatccttctatggttagaccgctttcgaatttcctcttgaaagctgcataattcttcactcaccttcgcaagttcttcaagagctgtactgagggcgccagaacagctcttgctgtcttcctcagaagtcctcaggtcaggccaggcctcacattccttttggttgtctgtagccaaaggatccaaaaaccctacttttgatttttttgttgctttttgttccttacacatttgatttcctccactgactaagctctgctctcttttattttcttttctcagaccatctttgtgattcgtccttataaattcactttgtcctaaatcggggtaatttggggaagattctatcactttctctggaatggtcttctcatggtaaagatcaatgatcttagcactttcattgatattgattttcctccaaagctttacttcccggcaaagctcttctattttcttctgcataatcttccattgactttcccattcctttctttcattgtcaaactggtccagtaattccatcttttccttatgccagttagtctctgtgttctcccactgcttatgtaggtccatggcaacagtgtaagtgtcagcaaagaagtgtttctgctcttctctgcctcctcttaactgtttcttggaagcttgaagttgttttatttgaagcagtctcacttgcctttaaaataaagcctgaaatattttagtgtttgggcttcttattgaatttggtcttggtaagatgagttgtatctttttaaagaaataagcagtcttcagtgtttttatagcattggttactacagaaattatacttcttttacttcttgtcttgaagggtgaacaaaataaacaaactgaaaatactacaatgaatggtaaatgatgaaagatttacagtacaaaaaacagtgtaaaaaggaagacaagtttaaatattgttgtgtaagaaagtgatgaaaataatacaagaatgagaataagtaaaatgataggctggaacatctgactcacggaaatgggctcctcggcgccgcggtcgtccgcagacttgggcacctcgaggcggtcgatgaaggtctgcagctccttgcggaaggccttcatctgagcgttgatgcggtagagcagctcgtgctcccggatgcggctgccgtcgtcctcctcgtccatgagtccgaacaggtccccgttggccacgtagatgcgcgcctcggtgatgatggtgctcgtgtcggcgatgagccggtcgatggtcttgcccaggcgctcggcctccgagcggatgtccttcatctgctgccgatcggagaagctcttgggccagggcccgggcgccgggtagaaggagcgagtgggcgtgaggcagcggatgttgcgcacctcctccgagtcgctctcgccgccgatgggcccttcgcgcttgcggtgcggaggccgcgagtcgtcgtcgctctccttcttgcccgcgtcgctctcggcgtcgctgtcgcgggggctgccgcggatgcccaggtgcgaggccaggtcgtagcgctgcatgttggacataagcacgcggttctcgtactgcagctgcatgaccttgccgctgagctcgttgatctgcaggcgcgccgccttcagctcctcctgcagggcctcggtcttggcgttgtcgtggtgccgcgcgctgtcgtggccgccggacttgtacttgtacttgttgagctccgccgtgatgcgcttgttctgctcctccaggtcggccacgttcctccgcagcagctccgtctcgtcttccaccagctgcaggtgctgccgcagctccgacagggattcgctctgctccctcatgagcgggttggccgagccgttgaagtcatcgcccctaaggtcgtccagttccgccttcaggcctctgttctccacctccagttcgacgattttcctgcccaggatgttggcttcttcctccaccagccttagccgtagcttgagctcggcctccctagtgctgggagggcctccggcttctcctttgggcaaaggactgtccagatccccataaaaggatctgtacttctggagctcgtgttcaaatctgtccttttctttatcaatcttggccattttctttctcatcaaagcggcttcttccttaacaaactgcagctggcacttcagatcttcattgtcctcctctgtgggagtctgttgagcctttttttcagattttggcaaatctttgcttcctcttctttttaaggataactctttcattttttccagttcattctgtaaagcttgctttgcaatttcaacttctatgagctgttgcctcagtttctcattttcatcttctgttgttgttctcttttcttccacattttctaattcatggtgaagtctcacagatacatcctttgcaaccttgaggtcctgctccaggctgcgcaacagctccccgtcgatttccccggtctgggcgtagcggagccttttgcgctcggctttgcggaggcggtactgcaggatccggcagtttttgttggctctctccaactcgtggcgcatttcctgcagttgacaggcatcctcctcgaagaaagtgtccctcatctcgtccatctcggttctcagctcatcgatctcgttcttgagagtctcgttttcctctcgcagcttctccatctcctcttgcatttcttcctgctcttggagctgctgcgggtgcggctgcgacgaagggggcgctgccgcctgcatgcccccgccgctcgcgctgccctctgcgctctgctgggggccctccgccgccgccgccattggggaggcggaggcgacggccagggtctcgcaaacggcaggggggccagacaccggggagctgcggctactgctgccgccgccgttcttagcgtgcatctgagccgcggccgccgccgctgccgcccgctccttcttgagatggaactggatgagctcagactgcagacatccttctttccagtagctccctccaccaccgctgccgccccccgcaacgccgcttccggagtttctgctgccggttcctggggttttgcccgcagaagaggaggatggagaaggggaggccccctccccgccgctgccgcccctctgctgagcgcgtacgcctttccctcgccagcccctgggcggcggcggctgcggagcgcccccctccctttccccggagccgccgccggctcctcctccttccccgccccctcctcccccttctccgagcggagggggttccccgagtttcgagggcacggactctagctcccgaggcggctcctcgggcggtccgggcctcctgccgcccaaagcggccagggtcgcggcgggggccgcttcagcaccagccacaggctggacagctcccggagcggcccctttgggcgccaggggcgtcgccttctcggccccacctccgcctcctcggatgctggcgggcggccccgtgcggctcccggtcttgttaccctgctgttgctgctgctgcagctgctgctgccgaacagaattgagtttagtgccggcccccactggggaccgggtggccgcgattgtctgtcgcagcgaactgtccctcggtctagcgggtgactgagctcgctgctgctttctgctgctgccctccgggtgcagacgagcctcagtggctgcagcggcgggagaagctgctgctgtggcaggggcagcgcccccgattggtggctgactcatggctatgaacctaccagatgcgatttggaagagcccattactagatcatcctcttccctcttcaccgccgccaaccttccttcctaagttctcagcagaggcgaggtttccaagtagctgaacaaatcaacagcactttccttctgatattccggggatctcagggtttattattgtgcctttctgcgccgaggaaagttcaacttcatattattgtatgcgactttccggctgagcatgactttgggctcgctcgccgcagttccacacccactcgatttctccaaacaatggcggtaacgtcaagattcagctgcccccagagcgggtgacttcccggcggtccgcggctgggctggagctgcagctctcagcaggctaacacgcgaggtaccaagctgggccagacgctccccaggaagtgcagagatgttcatgagctgacctcaccgaactgggcaggagagaaggcgggattgcaagggacgatagggtagaagtaaccaaagagaggttactttcaagaggaaagag

SEQ ID NO: 10929 - RNA, 6081 nt, Homo sapiens
  source 1..6081: mol_type = other RNA
ctgaatagctgggactacaggtgaccaccacaatgcctggctaattttttgtatttttagcagagagggggtttcaccgtgatgaaaccaggatggtctccatctcctgacctcgtgatccccccaccttggcctcccaaagtgctgggattacaggcaagagccaccgcgcccaccagttctaagttccgatacatgtacttgctacttaagaaaaacatgccgaatttaaagcaaatagtactgtaataaaaaaatctgattttcctgaaaatggtttaattttatgatgtaaatgcaaatcttagaagtaaaaacttttttcaaagaagacttttatcagactcaattagcagttaaatgggtagagagaggatgtcagtgtacgagaagccatatggagttttgggtggccaggagcaggaagtcaggcaggtttggcttcagttgtactacctagagatattttggaagaagctagagtgaactgtgtacatatatgagtttagatttcataagacacttagctttactggagttcactgcagaaaatgagggaaagaaaaatgttctcgatgtatacaaatgccacagacagttgtttttacacctactttatttgatagcttctaatggctgaaggagatttcaatatcaagtagttgtttgtcacaaatgtgcctaaaaataactttaaagatctttgtagggaagcagaaactcttaagtccagatgttttctcaggataactaaacctggtaaaatcacctatatagaagtaaataatattttatggccacatctgcaaaatgaaatatgatcatcttcattgtcgatataaaaacaaatgaaagttatgggtaatttttgataaaatgaattatacaaagcatcatttatatttttatatttggctttgggacataaggcaatatggagaacttatgtgacactgacacaaacacacacacacacacacacacacaaactcaagtactcctctctgcctcatccttattcctttctgagatcagcccataatatcagtaatcctctgctgaactaaaataatatttttgctccaaaagtctgctagggaaaacatctattaatatatgtttttaaatcaaatatttccagaaatgcttacaagtccctttaaatctagcaatgatagcataataaagggcatattctagggaagaaaatgcccacctaaagtagaaatttaccagttaaaaatcacaaaacatcaaaaactattttcaaggattatttccatttacctaataggtttttccatttaaaagttataaaatatttaaaaagagaaaacagaacattcaaataaccttagtttttcagttttacaatcaaggagttggactagatgctattttttttttctcagctctaactataattttagtcaacataagaagacgttaaaatgtgtcccactggttcattcaactgttaatagaaaaaagtggcttaaaattgtgaagtctgaaagtatagccattctaatttacagataacaaaggcaagtcctaggaagaaaagtgaccacccaagggcatccatccattcagagatcaagcaatgtcactgttttcaaatctgcctgatcatcaatattttgctttgttttgttttgttttattaatggttctggagtcccagtccctacccctggaaattttgctttagtaatatggggtgagatcagaaatttcattttttaaagagatcctcaatattctaaggaaccacagatcataccagactacttgggatacactggtggagaggaacagataggttgcacagtccttgggcaggctctccattgtcacacaacagcattttcctaacaggtccgtcattttatgacccagggttcctctttcctggtgttttctcccctctagctggaaagcatattatgagagtgatattacttggtgtctagtttacttttctttgatagcttcctgtggaaaaggatcttcctgaaggaaataagaattaaaagagtagatgtatagaccttagttaccatccaatacaaatcactctagacctttaattccacttaactaccgaaactgtccttacagtaaagtatgaatctagacatcaccatgctacagtcttgagcctttcaaggaagtctgcaatttgaaaattattttctttacctcaggtcatggggtacaatgaagtgaatttctctaaatggttcaaatacatcataaggagatggctcttggaatacatttggcataagaatttcttagtaaaagaaaagcttaaatagagttaatatctaataacataacataattggttttatatagtgacagtagagagcaaagttccttctaaaatcttccatttagaattccaagcccctcgacattcatatttctgtcagttttcaatatagattttatgtgttcactgtatgcaaactgtagccaaaatacacatttctattcctgatgctactgtggatgtcaaggtttagtttaagccttttttcggtagcaaactgtgagaagtataatttcagctttcaaagaaatattattcctgatcttccttgttagtaaaaaagtaacttagtttgttatctattaattttaaggaaaagattagaaaaaggaaaaaaataataaatgacttacctctaagtatgtatgactccatgttaaagcagctaaactaaaagcttaccacaacttaaagaaaaactaaaattcaacatcattcagtttctttttgcatcccatttaggaaatgtttgttgctgaggctgacaaaataaattcatcatttaatcatgtcatttataatgcagtctcatgatactgtctctgaggatcaaatattcagttaaagccatactagactaccaaataatatataaaacatttatgaacattttatgcttgctttacaaggctgatctattaaacttgtgacatttttatttaaaaagaataaacaagaatatcaatggtattattttatccttatatgggttaagaaattatttatgagttgtctttagaaatctaccaatgttagatgtgtgcataattcttctttttcattgtagctgggggccaaggaagtggtcaattaatatttgtactgcaaatgccttaagtggatacctattaaaaggtatacaaaatataaacagtactgcatattttcaaaacttttaaataaacacaaagaatatataggtatacatgttataatttcaaagtcaacactagcacataagtttttcatatctaaatacatactaggatacttcctatttcaacacatgcacctacaaacacatggccatgcacataaccttactttctgccacttgcaacaaagaatatacaatattgtacattgtttcaacttatattgtattggaaaactaatgaggatggcattaaaaaattctgatctaagaaatcaaaatgcaggaagataattattccttagattaaaaacactgaagactgatggaaagttaagattcaaattgcttgtcggaagagaacaggtccgcctgtaaacactcagaatgctctgtttgacaagtgggactagaacttctgtaatatagcaatccaggccaaagacttaaaccatcaatgcttcggatcgcagagaaatggtatagttgtgggtagttctccgcaaggcagggggtgcagatggagatctggatgcccatctggaggggagacgacgatttgctggtctagcaggtcgggaaaatccttttccatgtgaggcgttcactgacatggattcctctgttatctttttcggatctattccttgcttcacttcctgtcccccccacacagctgtcttttgctgaaactgttgttccatttggagcatttctaaatgctgacttaatgtggcaccaccactgacatcagaattacatttggtccaattatcctggaagcacttagaattttgcaatgcagactctgttgctgtctcataggttttcagcagcttttccacaacaccataatttgacctgggatcagctgacctcggacggccagacaaattactcggtctccagtcatgctcgtggagcatatttcgataactgcgaggacttaggtgtccctgcatttgtcttactaggcctgttgtggatttcttggtgggattatcaggcacattttccatgggcacaggcatgtgggcattggttttccaaataccggacacatcgttactttgtgatatgctacctgtgtgagtagatgaggtatcacagggcttgagatcctccgatgattttgagcagctgtgattttgctgtattgcctgacaatttctatctgttctaaatacagttctgttaaattcatcagtctttgctgccagcttctcattccttgtagtcctttcaaagccacaactgaaatttctaagtgggctactgctctctgctactgaggagctacagtcattacttacatgaagatcaggatgagatttagcagggtgatctgggatcaccatttcatattttggattactgggggtagagcaggttttctgaaaccacgaagtagaggggctcctttttgcacctatcccaatgtcacatgaccacatgctaagtccaacatcttcattacttggaggcttgctatctattttgacttctggtaccaaagaggaaaagatgataccatctttcgaagttttcccttcatttggatacaacatagacatctcttgttgtctcaaagggaagtgagggttgtaattccttttacttcgaccctcatggggcacccagctgttgtggtctaacctttccttccatctttcataggcttgttcagaatccgagctgggaaaatttcgagaggtgcttcttggaggaggaactggtggagtttcatttctttttaaatcgattgtatcaattccacattttttcgtagaattgctctggagcacattggtacagctcagattcttcctgtttttctgtttttctttttctaaactgattggaagaatgcactggtcattgttgatcatggggtccccatgaggtatattagttacatttggcatttcctggagaaaagaatctgacttcatccttctatggttagaccgctttcgaatttcctcttgaaagctgcataattcttcactcaccttcgcaagttcttcaagagctgtactgagggcgccagaacagctcttgctgtcttcctcagaagtcctcaggtcaggccaggcctcacattccttttggttgtctgtagccaaaggatccaaaaaccctacttttgatttttttgttgctttttgttccttacacatttgatttcctccactgactaagctctgctctcttttattttcttttctcagaccatctttgtgattcgtccttataaattcactttgtcctaaatcggggtaatttggggaagattctatcactttctctggaatggtcttctcatggtaaagatcaatgatcttagcactttcattgatattgattttcctccaaagctttacttcccggcaaagctcttctattttcttctgcataatcttccattgactttcccattcctttctttcattgtcaaactggtccagtaattccatcttttccttatgccagttagtctctgtgttctcccactgcttatgtaggtccatggcaacagtgtaagtgtcagcaaagaagtgtttctgctcttctctgcctcctcttaactgtttcttggaagcttgaagttgttttatttgaagcagtctcacttgcctttaaaataaagcctttcacactggggagaaatcctatggatgctcgaccactggtcaattagcagtggaagaaagtggatggctagctgtcttaaagagaaaagtctcagctcggtgaatctcgattctttacaagaaaaggggatgcaaaataagtccaaccattccacagagcagtactgacaagtccctttgaaaccttcaccacttttacaagtcaaaaagct

SEQ ID NO: 10930 - RNA, 2687 nt, Homo sapiens
  source 1..2687: mol_type = other RNA
ctgaatagctgggactacaggtgaccgccaccacgcctggctaatttttttgtatttttagtagagacggggtttcactgtgttagccaggatggtctcaatctcctgaccttgtgatccaccagcctcggcctcccaaagtgctgggactacaggcatgagccaccgtgcccagaatgttctgtttttgtttgtttgtttgtttgttttttgagacagggtctcgctctgtcactcaggctggagtgcagtggtgcaatcacggctcactgcagccttgacctcccaggctcacatgatcctcccacgacagcctctggagtgtcccctccactttctttcttaggggcccctcagggacatgtcagaggcctgagactacttgggggatgtctatgggccaggcaggctgccagcagctgagctgtccttgccctggggctcctctgcagtcagggagacaccaggcatgggcctggcttggatgcatcagtacttgactgcaaagacttaaaccacagacaggaaaggcgctgctgcagtctcgacggtcaaatgcagggccccctcagctgccatcccactgaggggcgaaggcccatcatctcccttcggctcggtaactgcctggcgtagcacaagggttctctttaaatccccagcaaatggagctgagtggaaattccgccccatattaccaggcacacgtctccttccactcctcactataccctgcccatgccacggccgccttctgagaataacgctgacagttccatggcccacagcccctctagttaacttgctgtgcacacggcagcccagccagaaacacgcagccaggtcggatattgggtgcattcagtcgtgaagcctgaggcttcctggctcccactgagcacagagaagtgttctgaaggacaggaagcagctggcctcactgctcttctcagacggctgatggagaaaagctcacagctgcctgcgccgctctgcctggacttgcatcctcggccccaccccttgcgcagcagtgaggccccccgagacactggtgcctgggcttgcggtaccgcagggctgctggacaacgggccagacgcagccccagtgtggatccagaggtctctctccgtagcaagccatggaagcacgacgggcactgtgctgagaaccctggtctgcacttctgacctggggctctggctgtgcggttctgctgagctcatccgagagtccacgcgtgcatggcggagacctgagtcagcggcagggccaccccgttatgggcaccccaaccccttattaggggtgttaatcagcacaaatgagcaactggctcatcagtcggtgcaggctgacaggtgcaggaaatacggagggcaggcggggtagggggcacggaatgcttcccaacatgagggcatctcaggccagcaggcggggcccagagacccagaagcaccacaactcccccgtgtccacaaggcactttatgcattcaaaaccaccgaattcacacccaggtttgctcagacagaggcccagaggcgaccccgctctggcgtggctaccacctgagcggctggcggccctggcccagctcggcctccgcgtaggcgtcatacagcaccttcaggtgcaacagcagctgctccaggttctcgccggtcaacgccgacagcacgatgacctcctgtcccaagtgatcccggagctgggacagattggcttgggcttcagggaggtcaatcttgtttgcgacgattgcgtggggcctcgcagacaggcccttttcatacatctccagttcatattttaaatcgtcaacttgagtccacggctcaggctgagaaagatccaccacgaacaagagaaagcggcagcgctcgatgtgcctgaggaaggcggaccccagacccctgttctggtgggcgcctcgtatgatgccggggatgtcggccacattccggcgtgggccaccgtcttgagctccaggtggagaactcgctgctgtcctggctgtccaggggtacaggtcacaggggcacggttgttgttggccaggaagaagcggttgcctttccctcctgccccgcccagcgcggcaatgtactcatctcccacgcaagacaggtcggccacaactctgcctccctccttcaccagcgtgcccacggggacccggatgtagaggacggcgccactgcgcccgaagcagtttttactccctccatcttctccactgaaaccctggtaccgcgacaggaccgacgacagggacttgacttgctggtcaactctcagaatgacgtgtccaccgttgcctccgtcccctccatcagggcctccaaactccttgcggggctcactgtggaagcagcttgccccagcgcctccgtttcctccacagacaagcactctccgatagtccacaaagtaccttttcagctttttctcagagagcagcttcttccccgggagttcctgatgcttggcgaggtccgcacggccgaccgagagcagcctgggagaagcccgctgtggcagtagccggctgggcttcaggccagcccatgtggacaaagcccaatgccccacgccctgaaacacggtcctcaatcttgctgagaaacaccttgcaggtgccatggccccggctcgggaaagcacgtcacttccggagc

SEQ ID NO: 10931 - RNA, 2544 nt, Homo sapiens
  source 1..2544: mol_type = other RNA
ctgaatagctgggactacaggtgaccgccaccacgcctggctaatttttttgtatttttagtagagacggggtttcactgtgttagccaggatggtctcaatctcctgaccttgtgatccaccagcctcggcctcccaaagtgctgggactacaggcatgagccaccgtgcccagaatgttctgtttttgtttgtttgtttgtttgttttttgagacagggtctcgctctgtcactcaggctggagtgcagtggtgcaatcacggctcactgcagccttgacctcccaggctcacatgatcctcccacgacagcctctggagtgtcccctccactttctttcttaggggcccctcagggacatgtcagaggcctgagactacttgggggatgtctatgggccaggcaggctgccagcagctgagctgtccttgccctggggctcctctgcagtcagggagacaccaggcatgggcctggcttggatgcatcagtacttgactgcaaagacttaaaccacagacaggaaaggcgctgctgcagtctcgacggtcaaatgcagggccccctcagctgccatcccactgaggggcgaaggcccatcatctcccttcggctcggtaactgcctggcgtagcacaagggttctctttaaatccccagcaaatggagctgagtggaaattccgccccatattaccaggcacacgtctccttccactcctcactataccctgcccatgccacggccgccttctgagaataacgctgacagttccatggcccacagcccctctagttaacttgctgtgcacacggcagcccagccagaaacacgcagccaggtcggatattgggtgcattcagtcgtgaagcctgaggcttcctggctcccactgagcacagagaagtgttctgaaggacaggaagcagctggcctcactgctcttctcagacggctgatggagaaaagctcacagctgcctgcgccgctctgcctggacttgcatcctcggccccaccccttgcgcagcagtgaggccccccgagacactggtgcctgggcttgcggtaccgcagggctgctggacaacgggccagacgcagccccagtgtggatccagaggtctctctccgtagcaagccatggaagcacgacgggcactgtgctgagaaccctggtctgcacttctgacctggggctctggctgtgcggttctgctgagctcatccgagagtccacgcgtgcatggcggagacctgagtcagcggcagggccaccccgttatgggcaccccaaccccttattaggggtgttaatcagcacaaatgagcaactggctcatcagtcggtgcaggctgacaggtgcaggaaatacggagggcaggcggggtagggggcacggaatgcttcccaacatgagggcatctcaggccagcaggcggggcccagagacccagaagcaccacaactcccccgtgtccacaaggcactttatgcattcaaaaccaccgaattcacacccaggtttgctcagacagaggcccagaggcgaccccgctctggcgtggctaccacctgagcggctggcggccctggcccagctcggcctccgcgtaggcgtcatacagcaccttcaggtgcaacagcagctgctccaggttctcgccggtcaacgccgacagcacgatgacctcctgtcccaagtgatcccggagctgggacagattggcttgggcttcagggaggtcaatcttgtttgcgacgattgcgtggggcctcgcagacaggcccttttcatacatctccagttcatattttaaatcgtcaacttgagtccacggctcaggctgagaaagatccaccacgaacaagagaaagcggcagcgctcgatgtgcctgaggaaggcggaccccagacccctgttctggtgggcgcctcgtatgatgccggggatgtcggccactgctatttgtaggtggccttcgtagtggacgatcccgacgtggggcttcagggtggtgaacgggtaggaagccacggcgggtctggcgtttgaaatggcccggagcagtgaggacttcccggcgttggggaatcccaccattccggcgtgggccaccgtcttgagctccaggtggagaactcgctgctgtcctggctgtccaggggtacaggtcacaggggcacggttgttgttggccaggaagaagcggttgcctttccctcctgccccgcccagcgcggcaatgtactcatctcccacgcaagacaggtcggccacaactctgcctccctccttcaccagcgtgcccacggggacccggatgtagaggacggcgccactgcgcccgaagcagtttttactccctccatcttctccactgaaaccctggtaccgcgacaggaccgacgacagggacttgacttgctggtcaacgaacccaccacacaggcctcgtgctttcacgcgaccgacatgtcagcttccctgacaggaaactctctgtgctccggctcgggaaagcacgtcacttccggagc

SEQ ID NO: 10932 - RNA, 2901 nt, Homo sapiens
  source 1..2901: mol_type = other RNA
ctgaatagctgggactacaggtgaccgccaccacgcctggctaatttttttgtatttttagtagagacggggtttcactgtgttagccaggatggtctcaatctcctgaccttgtgatccaccagcctcggcctcccaaagtgctgggactacaggcatgagccaccgtgcccagaatgttctgtttttgtttgtttgtttgtttgttttttgagacagggtctcgctctgtcactcaggctggagtgcagtggtgcaatcacggctcactgcagccttgacctcccaggctcacatgatcctcccacgacagcctctggagtgtcccctccactttctttcttaggggcccctcagggacatgtcagaggcctgagactacttgggggatgtctatgggccaggcaggctgccagcagctgagctgtccttgccctggggctcctctgcagtcagggagacaccaggcatgggcctggcttggatgcatcagtacttgactgcaaagacttaaaccacagacaggaaaggcgctgctgcagtctcgacggtcaaatgcagggccccctcagctgccatcccactgaggggcgaaggcccatcatctcccttcggctcggtaactgcctggcgtagcacaagggttctctttaaatccccagcaaatggagctgagtggaaattccgccccatattaccaggcacacgtctccttccactcctcactataccctgcccatgccacggccgccttctgagaataacgctgacagttccatggcccacagcccctctagttaacttgctgtgcacacggcagcccagccagaaacacgcagccaggtcggatattgggtgcattcagtcgtgaagcctgaggcttcctggctcccactgagcacagagaagtgttctgaaggacaggaagcagctggcctcactgctcttctcagacggctgatggagaaaagctcacagctgcctgcgccgctctgcctggacttgcatcctcggccccaccccttgcgcagcagtgaggccccccgagacactggtgcctgggcttgcggtaccgcagggctgctggacaacgggccagacgcagccccagtgtggatccagaggtctctctccgtagcaagccatggaagcacgacgggcactgtgctgagaaccctggtctgcacttctgacctggggctctggctgtgcggttctgctgagctcatccgagagtccacgcgtgcatggcggagacctgagtcagcggcagggccaccccgttatgggcaccccaaccccttattaggggtgttaatcagcacaaatgagcaactggctcatcagtcggtgcaggctgacaggtgcaggaaatacggagggcaggcggggtagggggcacggaatgcttcccaacatgagggcatctcaggccagcaggcggggcccagagacccagaagcaccacaactcccccgtgtccacaaggcactttatgcattcaaaaccaccgaattcacacccaggtttgctcagacagaggcccagaggcgaccccgctctggcgtggctaccacctgagcggctggcggccctggcccagctcggcctccgcgtaggcgtcatacagcaccttcaggtgcaacagcagctgctccaggttctcgccggtcaacgccgacagcacgatgacctcctgtcccaagtgatcccggagctgggacagattggcttgggcttcagggaggtcaatcttgtttgcgacgattgcgtggggcctcgcagacaggcccttttcatacatctccagttcatattttaaatcgtcaacttgagtccacggctcaggctgagaaagatccaccacgaacaagagaaagcggcagcgctcgatgtgcctgaggaaggcggaccccagacccctgttctggtgggcgcctcgtatgatgccggggatgtcggccactgctatttgtaggtggccttcgtagtggacgatcccgacgtggggcttcagggtggtgaacgggtaggaagccacggcgggtctggcgtttgaaatggcccggagcagtgaggacttcccggcgttggggaatcccaccattccggcgtgggccaccgtcttgagctccaggtggagaactcgctgctgtcctggctgtccaggggtacaggtcacaggggcacggttgttgttggccaggaagaagcggttgcctttccctcctgccccgcccagcgcggcaatgtactcatctcccacgcaagacaggtcggccacaactctgcctccctccttcaccagcgtgcccacggggacccggatgtagaggacggcgccactgcgcccgaagcagtttttactccctccatcttctccactgaaaccctggtaccgcgacaggaccgacgacagggacttgacttgctggtcaacgaacccaccacacaggcctcgtgctttcacgcgaccgacatgtcagcttccctgacaggaaactctctgtgctcctctcagaatgacgtgtccaccgttgcctccgtcccctccatcagggcctccaaactccttgcggggctcactgtggaagcagcttgccccagcgcctccgtttcctccacagacaagcactctccgatagtccacaaagtaccttttcagctttttctcagagagcagcttcttccccgggagttcctgatgcttggcgaggtccgcacggccgaccgagagcagcctgggagaagcccgctgtggcagtagccggctgggcttcaggccagcccatgtggacaaagcccaatgccccacgccctgaaacacggtcctcaatcttgctgagaaacaccttgcaggtgccatggccccggctcgggaaagcacgtcacttccggagc

SEQ ID NO: 10933 - RNA, 2918 nt, Homo sapiens
  source 1..2918: mol_type = other RNA
ctgaatagctgggactacaggtgaccgccaccacgcctggctaatttttttgtatttttagtagagacggggtttcactgtgttagccaggatggtctcaatctcctgaccttgtgatccaccagcctcggcctcccaaagtgctgggactacaggcatgagccaccgtgcccagaatgttctgtttttgtttgtttgtttgtttgttttttgagacagggtctcgctctgtcactcaggctggagtgcagtggtgcaatcacggctcactgcagccttgacctcccaggctcacatgatcctcccacgacagcctctggagtgtcccctccactttctttcttaggggcccctcagggacatgtcagaggcctgagactacttgggggatgtctatgggccaggcaggctgccagcagctgagctgtccttgccctggggctcctctgcagtcagggagacaccaggcatgggcctggcttggatgcatcagtacttgactgcaaagacttaaaccacagacaggaaaggcgctgctgcagtctcgacggtcaaatgcagggccccctcagctgccatcccactgaggggcgaaggcccatcatctcccttcggctcggtaactgcctggcgtagcacaagggttctctttaaatccccagcaaatggagctgagtggaaattccgccccatattaccaggcacacgtctccttccactcctcactataccctgcccatgccacggccgccttctgagaataacgctgacagttccatggcccacagcccctctagttaacttgctgtgcacacggcagcccagccagaaacacgcagccaggtcggatattgggtgcattcagtcgtgaagcctgaggcttcctggctcccactgagcacagagaagtgttctgaaggacaggaagcagctggcctcactgctcttctcagacggctgatggagaaaagctcacagctgcctgcgccgctctgcctggacttgcatcctcggccccaccccttgcgcagcagtgaggccccccgagacactggtgcctgggcttgcggtaccgcagggctgctggacaacgggccagacgcagccccagtgtggatccagaggtctctctccgtagcaagccatggaagcacgacgggcactgtgctgagaaccctggtctgcacttctgacctggggctctggctgtgcggttctgctgagctcatccgagagtccacgcgtgcatggcggagacctgagtcagcggcagggccaccccgttatgggcaccccaaccccttattaggggtgttaatcagcacaaatgagcaactggctcatcagtcggtgcaggctgacaggtgcaggaaatacggagggcaggcggggtagggggcacggaatgcttcccaacatgagggcatctcaggccagcaggcggggcccagagacccagaagcaccacaactcccccgtgtccacaaggcactttatgcattcaaaaccaccgaattcacacccaggtttgctcagacagaggcccagaggcgaccccgctctggcgtggctaccacctgagcggctggcggccctggcccagctcggcctccgcgtaggcgtcatacagcaccttcaggtgcaacagcagctgctccaggttctcgccggtcaacgccgacagcacgatgacctcctgtcccaagtgatcccggagctgggacagattggcttgggcttcagggaggtcaatcttgtttgcgacgattgcgtggggcctcgcagacaggcccttttcatacatctccagttcatattttaaatcgtcaacttgagtccacggctcaggctgagaaagatccaccacgaacaagagaaagcggcagcgctcgatgtgcctgaggaaggcggaccccagacccctgttctggtgggcgcctcgtatgatgccggggatgtcggccactgctatttgtaggtggccttcgtagtggacgatcccgacgtggggcttcagggtggtgaacgggtaggaagccacggcgggtctggcgtttgaaatggcccggagcagtgaggacttcccggcgttggggaatcccaccattccggcgtgggccaccgtcttgagctccaggtggagaactcgctgctgtcctggctgtccaggggtacaggtcacaggggcacggttgttgttggccaggaagaagcggttgcctttccctcctgccccgcccagcgcggcaatgtactcatctcccacgcaagacaggtcggccacaactctgcctccctccttcaccagcgtgcccacggggacccggatgtagaggacggcgccactgcgcccgaagcagtttttactccctccatcttctccactgaaaccctggtaccgcgacaggaccgacgacagggacttgacttgctggtcaactctcagaatgacgtgtccaccgttgcctccgtcccctccatcagggcctccaaactccttgcggggctcactgtggaagcagcttgccccagcgcctccgtttcctccacagacaagcactctccgatagtccacaaagtaccttttcagctttttctcagagagcagcttcttccccgggagttcctgatgcttggcgaggtccgcacggccgaccgagagcagcctgggagaagcccgctgtggcagtagccggctgggcttcaggccagcccatgtggacaaagcccaatgccccacgccctgaaacacggtcctcaatcttgctgagaaacaccttgcaggtgccatggccccataagatgtgtcataagtctcaatacattgagaagaaatcatagtcagtcctccgtatctgtggggtcaacaaacctcacgtcaaaaatatcggctcgggaaagcacgtcacttccggagc

SEQ ID NO: 10934 - RNA, 4888 nt, Homo sapiens
  source 1..4888: mol_type = other RNA
ctgaatagctgggactacaggtgaccgccaccacgcctggctaatttttttgtatttttagtagagacggggtttcactgtgttagccaggatggtctcaatctcctgaccttgtgatccaccagcctcggcctcccaaagtgctgggactacaggcatgagccaccgtgcccagaatgttctgtttttgtttgtttgtttgtttgttttttgagacagggtctcgctctgtcactcaggctggagtgcagtggtgcaatcacggctcactgcagccttgacctcccaggctcacatgatcctcccacgacagcctctggagtgtcccctccactttctttcttaggggcccctcagggacatgtcagaggcctgagactacttgggggatgtctatgggccaggcaggctgccagcagctgagctgtccttgccctggggctcctctgcagtcagggagacaccaggcatgggcctggcttggatgcatcagtacttgactgcaaagacttaaaccacagacaggaaaggcgctgctgcagtctcgacggtcaaatgcagggccccctcagctgccatcccactgaggggcgaaggcccatcatctcccttcggctcggtaactgcctggcgtagcacaagggttctctttaaatccccagcaaatggagctgagtggaaattccgccccatattaccaggcacacgtctccttccactcctcactataccctgcccatgccacggccgccttctgagaataacgctgacagttccatggcccacagcccctctagttaacttgctgtgcacacggcagcccagccagaaacacgcagccaggtcggatattgggtgcattcagtcgtgaagcctgaggcttcctggctcccactgagcacagagaagtgttctgaaggacaggaagcagctggcctcactgctcttctcagacggctgatggagaaaagctcacagctgcctgcgccgctctgcctggacttgcatcctcggccccaccccttgcgcagcagtgaggccccccgagacactggtgcctgggcttgcggtaccgcagggctgctggacaacgggccagacgcagccccagtgtggatccagaggtctctctccgtagcaagccatggaagcacgacgggcactgtgctgagaaccctggtctgcacttctgacctggggctctggctgtgcggttctgctgagctcatccgagagtccacgcgtgcatggcggagacctgagtcagcggcagggccaccccgttatgggcaccccaaccccttattaggggtgttaatcagcacaaatgagcaactggctcatcagtcggtgcaggctgacaggtgcaggaaatacggagggcaggcggggtagggggcacggaatgcttcccaacatgagggcatctcaggccagcaggcggggcccagagacccagaagcaccacaactcccccgtgtccacaaggcactttatgcattcaaaaccaccgaattcacacccaggtttgctcagacagaggcccagaggcgaccccgctctggcgtggctaccacctgagcggctggcggccctggcccagctcggcctccgcgtaggcgtcatacagcaccttcaggtgcaacagcagctgctccaggttctcgccggtcaacgccgacagcacgatgacctcctgtcccaagtgatcccggagctgggacagattggcttgggcttcagggaggtcaatcttgtttgcgacgattgcgtggggcctcgcagacaggcccttttcatacatctccagttcatattttaaatcgtcaacttgagtccacggctcaggctgagaaagatccaccacgaacaagagaaagcggcagcgctcgatgtgcctgaggaaggcggaccccagacccctgttctggtgggcgcctcgtatgatgccggggatgtcggccactgctatttgtaggtggccttcgtagtggacgatcccgacgtggggcttcagggtggtgaacgggtaggaagccacggcgggtctggcgtttgaaatggcccggagcagtgaggacttcccggcgttggggaatcccaccattccggcgtgggccaccgtcttgagctccaggtggagaactcgctgctgtcctggctgtccaggggtacaggtcacaggggcacggttgttgttggccaggaagaagcggttgcctttccctcctgccccgcccagcgcggcaatgtactcatctcccacgcaagacaggtcggccacaactctgcctccctccttcaccagcgtgcccacggggacccggatgtagaggacggcgccactgcgcccgaagcagtttttactccctccatcttctccactgaaaccctggtaccgcgacaggaccgacgacagggacttgacttgctggtcaactctcagaatgacgtgtccaccgttgcctccgtcccctccatcagggcctccaaactccttgcggggctcactgtggaagcagcttgccccagcgcctccgtttcctccacagacaagcactctccgatagtccacaaagtaccttttcagctttttctcagagagcagcttcttccccgggagttcctgatgcttggcgaggtccgcacggccgaccgagagcagcctgggagaagcccgctgtggcagtagccggctgggcttcaggccagcccatgtggacaaagcccaatgccccacgccctgaaacacggtcctcaatcttgctgagaaacaccttgcaggtgccatggccccataagatgtgtcataagtctcaatacattgagaagaaatcatagtcagtcctccgtatctgtggggtcaacaaacctcacgtcaaaaatatctggaaaacaaacaaaaaaaccagtaacaatacaacaatttttttaatttaaaaaataaagtataacagctatttacatagcatttacattgtattgtactataaataatctagagattacttgaagtatacagaaaggcccggtacagtggctcacacctgtaatcccagcagtttgagaggccaaggcaggagaaaaacttgaggccaggaatttgagaacagcctgggcaaaatagcgagaccttgtgtctaccaaaaaaaaaaaaaaaaaaaaaaaattagctgattagctggacatggtggtgcatgcctataataccagctacttaggaggctaaggtgggaggatcacttaagcccaggagttggaggctgcagtgaaccatgatcacacactgcactccagcctgtgtgacagagcttctgtggtggggctggggggaagtatatgaataccaaccacagggtctattctcggaattaaattggaagtcaatagctagaaaatatctaggaaaatcccaaatacctgcaaatcaaacaagcttcttctaaataatccataggccaaagaagaaatcaaaagagaaattacaaaatgttttgaactgaattataatggaaatgcaaaataccagaattttttttttttttttttgagacagtctcgcactgtcgcccaggctggagtgcagtggtgtgatctcggcccactgaaagttctgcctcccgggttcacgccattctcctgcctcagcctcccgagtagctgggactacaggcgcccgccaccatgaaataccagaatttaagagatgcagctagagtagtgtttagaaggaaacttacagctctaatggctaccttggtaaagaagaaagatctaaaatcagtaacctaaggctccaaatcaagaaaccagaaagagcaaagtaagcgtcgagtagaaggaggagaataatacagagcagaaataaagagacaacaataacatgtaacagaaaaaaacaggttcactgaaaagacaagctaactaacacacttctagcctgatcaggaaaacgagagagcgcaaacctccactgtcaggaatgttcaacgggttatcaggacacaccttacagacagccagagggcaagagaatgctgggaacgacttcatgccagcaaattcagtaacaaattcaacttacatgaaatggacaaatttcttgaaaaaggcaacttattaaagaaacacaagaataaacaatctagaatagccctgtatctactcaataagttaaatttcttataaaagaacactccccaaaggaaaactctagctcggcttgttttcctggtaaattccatgtaacattccaggaagaaacagtgccaatcttacacaagctttttcagaaaatagaggaagtgagatcactatccaactcatcctatgaggctagtaccaaaatctgacactaagaaaaaataaaattatagaccatacccctcatgaatatagatgcaaataactcttaacaaaatattacccaattgaatccagcagttcagaaaggatcacacatcaagacctagtaggggtaatctcagaacacaaggccacatcaagcagtcaaaactcagcccaggcacttcactatatcaacaggtggtaccaccgtctcaacacccactcatgaggaggaaaacaaaacatctcagcaaactgggaacagacgggaacatcttcgccctgataagggcactacgtagggccggccgacagctaatcacatttaatgaagaaatactgaatggttacctcccaagatggagaaaaagggcctccacacataccactgctatgcaacaatgtcctttcacacactgaaataaagggggaaaaaaggaagaagtaaaactgtccctgtttacagaagagaggacagagttccacagagaatcccagggaaggctgggcacggtggctcatgcctgtaatcccagcactt

SEQ ID NO: 10935 - RNA, 4833 nt, Homo sapiens
  source 1..4833: mol_type = other RNA
ctgaatagctgggactacaggtgaccgccaccacgcctggctaatttttttgtatttttagtagagacggggtttcactgtgttagccaggatggtctcaatctcctgaccttgtgatccaccagcctcggcctcccaaagtgctgggactacaggcatgagccaccgtgcccagaatgttctgtttttgtttgtttgtttgtttgttttttgagacagggtctcgctctgtcactcaggctggagtgcagtggtgcaatcacggctcactgcagccttgacctcccaggctcacatgatcctcccacgacagcctctggagtgtcccctccactttctttcttaggggcccctcagggacatgtcagaggcctgagactacttgggggatgtctatgggccaggcaggctgccagcagctgagctgtccttgccctggggctcctctgcagtcagggagacaccaggcatgggcctggcttggatgcatcagtacttgactgcaaagacttaaaccacagacaggaaaggcgctgctgcagtctcgacggtcaaatgcagggccccctcagctgccatcccactgaggggcgaaggcccatcatctcccttcggctcggtaactgcctggcgtagcacaagggttctctttaaatccccagcaaatggagctgagtggaaattccgccccatattaccaggcacacgtctccttccactcctcactataccctgcccatgccacggccgccttctgagaataacgctgacagttccatggcccacagcccctctagttaacttgctgtgcacacggcagcccagccagaaacacgcagccaggtcggatattgggtgcattcagtcgtgaagcctgaggcttcctggctcccactgagcacagagaagtgttctgaaggacaggaagcagctggcctcactgctcttctcagacggctgatggagaaaagctcacagctgcctgcgccgctctgcctggacttgcatcctcggccccaccccttgcgcagcagtgaggccccccgagacactggtgcctgggcttgcggtaccgcagggctgctggacaacgggccagacgcagccccagtgtggatccagaggtctctctccgtagcaagccatggaagcacgacgggcactgtgctgagaaccctggtctgcacttctgacctggggctctggctgtgcggttctgctgagctcatccgagagtccacgcgtgcatggcggagacctgagtcagcggcagggccaccccgttatgggcaccccaaccccttattaggggtgttaatcagcacaaatgagcaactggctcatcagtcggtgcaggctgacaggtgcaggaaatacggagggcaggcggggtagggggcacggaatgcttcccaacatgagggcatctcaggccagcaggcggggcccagagacccagaagcaccacaactcccccgtgtccacaaggcactttatgcattcaaaaccaccgaattcacacccaggtttgctcagacagaggcccagaggcgaccccgctctggcgtggctaccacctgagcggctggcggccctggcccagctcggcctccgcgtaggcgtcatacagcaccttcaggtgcaacagcagctgctccaggttctcgccggtcaacgccgacagcacgatgacctcctgtcccaagtgatcccggagctgggacagattggcttgggcttcagggaggtcaatcttgtttgcgacgattgcgtggggcctcgcagacaggcccttttcatacatctccagttcatattttaaatcgtcaacttgagtccacggctcaggctgagaaagatccaccacgaacaagagaaagcggcagcgctcgatgtgcctgaggaaggcggaccccagacccctgttctggtgggcgcctcgtatgatgccggggatgtcggccactgctatttgtaggtggccttcgtagtggacgatcccgacgtggggcttcagggtggtgaacgggtaggaagccacggcgggtctggcgtttgaaatggcccggagcagtgaggacttcccggcgttggggaatcccaccattccggcgtgggccaccgtcttgagctccaggtggagaactcgctgctgtcctggctgtccaggggtacaggtcacaggggcacggttgttgttggccaggaagaagcggttgcctttccctcctgccccgcccagcgcggcaatgtactcatctcccacgcaagacaggtcggccacaactctgcctccctccttcaccagcgtgcccacggggacccggatgtagaggacggcgccactgcgcccgaagcagtttttactccctccatcttctccactgaaaccctggtaccgcgacaggaccgacgacagggacttgacttgctggtcaactctcagaatgacgtgtccaccgttgcctccgtcccctccatcagggcctccaaactccttgcggggctcactgtggaagcagcttgccccagcgcctccgtttcctccacagacaagcactctccgatagtccacaaagtaccttttcagctttttctcagagagcagcttcttccccgggagttcctgatgcttggcgaggtccgcacggccgaccgagagcagcctgggagaagcccgctgtggcagtagccggctgggcttcaggccagcccatgtggacaaagcccaatgccccacgccctgaaacacggtcctcaatcttgctgagaaacaccttgcaggtgccatggccccctctcggccctgggtcacgtcttgccctctgacccgtcagcctatctgtgacttgggagcaggatttctgtacaaaggatttaaaacatgaaatcttccacaacactggacacatcctcttatggaatagcaaggttccgctcaacgaaaatattaaaaaggaaatctgaagtgcaagtcaaaatttcttgaaaagaaaaacacccatttattaaaatgttatcaagagtgttatcctgtgtaattttaaagttgttacattggaacacaagaatattaaacatggggcatagcggctaagcacccaggctctggaaagtaactctaagggaaggccatccacctgtgtggcctcggcctcctcacacggctgggtgaggacgggctgagctgatccacacggctgcacaaccgcggccctggctgtggcaccgatagaatgagaagaacacacttggcccctgctcctggctcctgacacagagctctcagaacgctggtaatttcctgagtgacaggggcgataggggtgcctgacacagagctcctaaatcccttggacttcccaggtgacaggagagtcttctgttctaatgaggcacctcttggtgggctcctggatggccttgggagggggctggtcatcataaagaccaagccacgatgagaagcctggacctttcggccccacccccaccctccaaaaagggcagaggggctggaggctgagttcataactgatcatgtctccatgatgaggcctccatggaaatcctggaactaggggctctggaaagctttcagtttggtgaactcatccccgtgctgtaaggccagccacacaactccctggggacaaaggctcctatgcttaggaccctctgggcctcgcccgtgcccctcctcacccagctgcctgcctgtgcccgctgtggcatcctttatagtaaactggcaatgcaaaccaagtgccttcctgagttctgtgagccactaccgcaaatcatcaaacctgaaggggtcgtaggaactcccaatgtgtagccaagatggacagaagtgtgggtaccccagggacccactacttgcaattagcatctgaagtggggggtgactgagcccctaacgctggggtccctgataaccgcggcagggtcagactgaactgaattacaggatgcctggctggtgtctgcagaggactggcgaattgttggtgtggaaaacccacacatttggtgcctgatgtgtagtgtgggtggaaatatccccggagcgacagggttggcacagctgcagactctaagtgccagctactgtcactctcaaagcctcatttaagctgtcactcattcaacaagccgctcatgacagccggctaccttgcaggtgccaagggcacagtgaggaagtcctgaccctgccctccaggagaggacagcccctctcccttcaccatgagcacaaatacctgcctgctcccagagctccccagtcttcagcaggtcgcacaggagggaccttacaaggtgctccccatcctgactacaaaagatgtgtacagaaggggccccagtggacggctgaaaactcaacacggggccagagcgggagcacaacgaggggacaccgcctgcctcctccctcgcagtgcctcggacgcctccctctccccagcctcactcctctgaaaaggtgccacctcctttgggggggtcactatctctgtggggtccttggccattctgctttaattctgaggcaatcacagttacagaaaagctggaagaagagtacaaagaacttcctcctgaatcacttaagagtcagtcgccgactggacttccctgcacccagaacagtccatgtgtgtttcctagagaaaatggtgtcccctccagaaccagggtgtcattgagactggccatgaccgacagcccctcccacgtgggccccggtctcagcagtgcctctccctgtaggaaagtctgcgtccctatcccggctgcctgcagctgccacaccttgtccagctc

SEQ ID NO: 10936 - RNA, 2826 nt, Homo sapiens
  source 1..2826: mol_type = other RNA
ctgaatagctgggactacaggtgaccgccaccacgcctggctaatttttttgtatttttagtagagacggggtttcactgtgttagccaggatggtctcaatctcctgaccttgtgatccaccagcctcggcctcccaaagtgctgggactacaggcatgagccaccgtgcccagaatgttctgtttttgtttgtttgtttgtttgttttttgagacagggtctcgctctgtcactcaggctggagtgcagtggtgcaatcacggctcactgcagccttgacctcccaggctcacatgatcctcccacgacagcctctggagtgtcccctccactttctttcttaggggcccctcagggacatgtcagaggcctgagactacttgggggatgtctatgggccaggcaggctgccagcagctgagctgtccttgccctggggctcctctgcagtcagggagacaccaggcatgggcctggcttggatgcatcagtacttgactgcaaagacttaaaccacagacaggaaaggcgctgctgcagtctcgacggtcaaatgcagggccccctcagctgccatcccactgaggggcgaaggcccatcatctcccttcggctcggtaactgcctggcgtagcacaagggttctctttaaatccccagcaaatggagctgagtggaaattccgccccatattaccaggcacacgtctccttccactcctcactataccctgcccatgccacggccgccttctgagaataacgctgacagttccatggcccacagcccctctagttaacttgctgtgcacacggcagcccagccagaaacacgcagccaggtcggatattgggtgcattcagtcgtgaagcctgaggcttcctggctcccactgagcacagagaagtgttctgaaggacaggaagcagctggcctcactgctcttctcagacggctgatggagaaaagctcacagctgcctgcgccgctctgcctggacttgcatcctcggccccaccccttgcgcagcagtgaggccccccgagacactggtgcctgggcttgcggtaccgcagggctgctggacaacgggccagacgcagccccagtgtggatccagaggtctctctccgtagcaagccatggaagcacgacgggcactgtgctgagaaccctggtctgcacttctgacctggggctctggctgtgcggttctgctgagctcatccgagagtccacgcgtgcatggcggagacctgagtcagcggcagggccaccccgttatgggcaccccaaccccttattaggggtgttaatcagcacaaatgagcaactggctcatcagtcggtgcaggctgacaggtgcaggaaatacggagggcaggcggggtagggggcacggaatgcttcccaacatgagggcatctcaggccagcaggcggggcccagagacccagaagcaccacaactcccccgtgtccacaaggcactttatgcattcaaaaccaccgaattcacacccaggtttgctcagacagaggcccagaggcgaccccgctctggcgtggctaccacctgagcggctggcggccctggcccagctcggcctccgcgtaggcgtcatacagcaccttcaggtgcaacagcagctgctccaggttctcgccggtcaacgccgacagcacgatgacctcctgtcccaagtgatcccggagctgggacagattggcttgggcttcagggaggtcaatcttgtttgcgacgattgcgtggggcctcgcagacaggcccttttcatacatctccagttcatattttaaatcgtcaacttgagtccacggctcaggctgagaaagatccaccacgaacaagagaaagcggcagcgctcgatgtgcctgaggaaggcggaccccagacccctgttctggtgggcgcctcgtatgatgccggggatgtcggccactgctatttgtaggtggccttcgtagtggacgatcccgacgtggggcttcagggtggtgaacgggtaggaagccacggcgggtctggcgtttgaaatggcccggagcagtgaggacttcccggcgttggggaatcccaccattccggcgtgggccaccgtcttgagctccaggtggagaactcgctgctgtcctggctgtccaggggtacaggtcacaggggcacggttgttgttggccaggaagaagcggttgcctttccctcctgccccgcccagcgcggcaatgtactcatctcccacgcaagacaggtcggccacaactctgcctccctccttcaccagcgtgcccacggggacccggatgtagaggacggcgccactgcgcccgaagcagtttttactccctccatcttctccactgaaaccctggtaccgcgacaggaccgacgacagggacttgacttgctggtcaactctcagaatgacgtgtccaccgttgcctccgtcccctccatcagggcctccaaactccttgcggggctcactgtggaagcagcttgccccagcgcctccgtttcctccacagacaagcactctccgatagtccacaaagtaccttttcagctttttctcagagagcagcttcttccccgggagttcctgatgcttggcgaggtccgcacggccgaccgagagcagcctgggagaagcccgctgtggcagtagccggctgggcttcaggccagcccatgtggacaaagcccaatgccccacgccctgaaacacggtcctcaatcttgctgagaaacaccttgcaggtgccatggccccggctcgggaaagcacgtcacttccggagc

SEQ ID NO: 10937 - RNA, 4983 nt, Homo sapiens
  source 1..4983: mol_type = other RNA
ctgaatagctgggactacaggtgaccgccaccacgcctggctaatttttttgtatttttagtagagacggggtttcactgtgttagccaggatggtctcaatctcctgaccttgtgatccaccagcctcggcctcccaaagtgctgggactacaggcatgagccaccgtgcccagaatgttctgtttttgtttgtttgtttgtttgttttttgagacagggtctcgctctgtcactcaggctggagtgcagtggtgcaatcacggctcactgcagccttgacctcccaggctcacatgatcctcccacgacagcctctggagtgtcccctccactttctttcttaggggcccctcagggacatgtcagaggcctgagactacttgggggatgtctatgggccaggcaggctgccagcagctgagctgtccttgccctggggctcctctgcagtcagggagacaccaggcatgggcctggcttggatgcatcagtacttgactgcaaagacttaaaccacagacaggaaaggcgctgctgcagtctcgacggtcaaatgcagggccccctcagctgccatcccactgaggggcgaaggcccatcatctcccttcggctcggtaactgcctggcgtagcacaagggttctctttaaatccccagcaaatggagctgagtggaaattccgccccatattaccaggcacacgtctccttccactcctcactataccctgcccatgccacggccgccttctgagaataacgctgacagttccatggcccacagcccctctagttaacttgctgtgcacacggcagcccagccagaaacacgcagccaggtcggatattgggtgcattcagtcgtgaagcctgaggcttcctggctcccactgagcacagagaagtgttctgaaggacaggaagcagctggcctcactgctcttctcagacggctgatggagaaaagctcacagctgcctgcgccgctctgcctggacttgcatcctcggccccaccccttgcgcagcagtgaggccccccgagacactggtgcctgggcttgcggtaccgcagggctgctggacaacgggccagacgcagccccagtgtggatccagaggtctctctccgtagcaagccatggaagcacgacgggcactgtgctgagaaccctggtctgcacttctgacctggggctctggctgtgcggttctgctgagctcatccgagagtccacgcgtgcatggcggagacctgagtcagcggcagggccaccccgttatgggcaccccaaccccttattaggggtgttaatcagcacaaatgagcaactggctcatcagtcggtgcaggctgacaggtgcaggaaatacggagggcaggcggggtagggggcacggaatgcttcccaacatgagggcatctcaggccagcaggcggggcccagagacccagaagcaccacaactcccccgtgtccacaaggcactttatgcattcaaaaccaccgaattcacacccaggtttgctcagacagaggcccagaggcgaccccgctctggcgtggctaccacctgagcggctggcggccctggcccagctcggcctccgcgtaggcgtcatacagcaccttcaggtgcaacagcagctgctccaggttctcgccggtcaacgccgacagcacgatgacctcctgtcccaagtgatcccggagctgggacagattggcttgggcttcagggaggtcaatcttgtttgcgacgattgcgtggggcctcgcagacaggcccttttcatacatctccagttcatattttaaatcgtcaacttgagtccacggctcaggctgagaaagatccaccacgaacaagagaaagcggcagcgctcgatgtgcctgaggaaggcggaccccagacccctgttctggtgggcgcctcgtatgatgccggggatgtcggccactgctatttgtaggtggccttcgtagtggacgatcccgacgtggggcttcagggtggtgaacgggtaggaagccacggcgggtctggcgtttgaaatggcccggagcagtgaggacttcccggcgttggggaatcccaccattccggcgtgggccaccgtcttgagctccaggtggagaactcgctgctgtcctggctgtccaggggtacaggtcacaggggcacggttgttgttggccaggaagaagcggttgcctttccctcctgccccgcccagcgcggcaatgtactcatctcccacgcaagacaggtcggccacaactctgcctccctccttcaccagcgtgcccacggggacccggatgtagaggacggcgccactgcgcccgaagcagtttttactccctccatcttctccactgaaaccctggtaccgcgacaggaccgacgacagggacttgacttgctggtcaactctcagaatgacgtgtccaccgttgcctccgtcccctccatcagggcctccaaactccttgcggggctcactgtggaagcagcttgccccagcgcctccgtttcctccacagacaagcactctccgatagtccacaaagtaccttttcagctttttctcagagagcagcttcttccccgggagttcctgatgcttggcgaggtccgcacggccgaccgagagcagcctgggagaagcccgctgtggcagtagccggctgggcttcaggccagcccatgtggacaaagcccaatgccccacgccctgaaacacggtcctcaatcttgctgagaaacaccttgcaggtgccatggcccctacagaagtcaaattggcaaaatgagatacttggtttaatgctgggcatgaaacagaaactgaagacgagggcctcatgcagcaggtctttgtgcacgtttctgaaacaaacaagtgaactgatgaatccgattttcctggtcactcaccctctcggccctgggtcacgtcttgccctctgacccgtcagcctatctgtgacttgggagcaggatttctgtacaaaggatttaaaacatgaaatcttccacaacactggacacatcctcttatggaatagcaaggttccgctcaacgaaaatattaaaaaggaaatctgaagtgcaagtcaaaatttcttgaaaagaaaaacacccatttattaaaatgttatcaagagtgttatcctgtgtaattttaaagttgttacattggaacacaagaatattaaacatggggcatagcggctaagcacccaggctctggaaagtaactctaagggaaggccatccacctgtgtggcctcggcctcctcacacggctgggtgaggacgggctgagctgatccacacggctgcacaaccgcggccctggctgtggcaccgatagaatgagaagaacacacttggcccctgctcctggctcctgacacagagctctcagaacgctggtaatttcctgagtgacaggggcgataggggtgcctgacacagagctcctaaatcccttggacttcccaggtgacaggagagtcttctgttctaatgaggcacctcttggtgggctcctggatggccttgggagggggctggtcatcataaagaccaagccacgatgagaagcctggacctttcggccccacccccaccctccaaaaagggcagaggggctggaggctgagttcataactgatcatgtctccatgatgaggcctccatggaaatcctggaactaggggctctggaaagctttcagtttggtgaactcatccccgtgctgtaaggccagccacacaactccctggggacaaaggctcctatgcttaggaccctctgggcctcgcccgtgcccctcctcacccagctgcctgcctgtgcccgctgtggcatcctttatagtaaactggcaatgcaaaccaagtgccttcctgagttctgtgagccactaccgcaaatcatcaaacctgaaggggtcgtaggaactcccaatgtgtagccaagatggacagaagtgtgggtaccccagggacccactacttgcaattagcatctgaagtggggggtgactgagcccctaacgctggggtccctgataaccgcggcagggtcagactgaactgaattacaggatgcctggctggtgtctgcagaggactggcgaattgttggtgtggaaaacccacacatttggtgcctgatgtgtagtgtgggtggaaatatccccggagcgacagggttggcacagctgcagactctaagtgccagctactgtcactctcaaagcctcatttaagctgtcactcattcaacaagccgctcatgacagccggctaccttgcaggtgccaagggcacagtgaggaagtcctgaccctgccctccaggagaggacagcccctctcccttcaccatgagcacaaatacctgcctgctcccagagctccccagtcttcagcaggtcgcacaggagggaccttacaaggtgctccccatcctgactacaaaagatgtgtacagaaggggccccagtggacggctgaaaactcaacacggggccagagcgggagcacaacgaggggacaccgcctgcctcctccctcgcagtgcctcggacgcctccctctccccagcctcactcctctgaaaaggtgccacctcctttgggggggtcactatctctgtggggtccttggccattctgctttaattctgaggcaatcacagttacagaaaagctggaagaagagtacaaagaacttcctcctgaatcacttaagagtcagtcgccgactggacttccctgcacccagaacagtccatgtgtgtttcctagagaaaatggtgtcccctccagaaccagggtgtcattgagactggccatgaccgacagcccctcccacgtgggccccggtctcagcagtgcctctccctgtaggaaagtctgcgtccctatcccggctgcctgcagctgccacaccttgtccagctc

SEQ ID NO: 10938 - RNA, 2818 nt, Homo sapiens
  source 1..2818: mol_type = other RNA
ctgaatagctgggactacaggtgaccgccaccacgcctggctaatttttttgtatttttagtagagacggggtttcactgtgttagccaggatggtctcaatctcctgaccttgtgatccaccagcctcggcctcccaaagtgctgggactacaggcatgagccaccgtgcccagaatgttctgtttttgtttgtttgtttgtttgttttttgagacagggtctcgctctgtcactcaggctggagtgcagtggtgcaatcacggctcactgcagccttgacctcccaggctcacatgatcctcccacgacagcctctggagtgtcccctccactttctttcttaggggcccctcagggacatgtcagaggcctgagactacttgggggatgtctatgggccaggcaggctgccagcagctgagctgtccttgccctggggctcctctgcagtcagggagacaccaggcatgggcctggcttggatgcatcagtacttgactgcaaagacttaaaccacagacaggaaaggcgctgctgcagtctcgacggtcaaatgcagggccccctcagctgccatcccactgaggggcgaaggcccatcatctcccttcggctcggtaactgcctggcgtagcacaagggttctctttaaatccccagcaaatggagctgagtggaaattccgccccatattaccaggcacacgtctccttccactcctcactataccctgcccatgccacggccgccttctgagaataacgctgacagttccatggcccacagcccctctagttaacttgctgtgcacacggcagcccagccagaaacacgcagccaggtcggatattgggtgcattcagtcgtgaagcctgaggcttcctggctcccactgagcacagagaagtgttctgaaggacaggaagcagctggcctcactgctcttctcagacggctgatggagaaaagctcacagctgcctgcgccgctctgcctggacttgcatcctcggccccaccccttgcgcagcagtgaggccccccgagacactggtgcctgggcttgcggtaccgcagggctgctggacaacgggccagacgcagccccagtgtggatccagaggtctctctccgtagcaagccatggaagcacgacgggcactgtgctgagaaccctggtctgcacttctgacctggggctctggctgtgcggttctgctgagctcatccgagagtccacgcgtgcatggcggagacctgagtcagcggcagggccaccccgttatgggcaccccaaccccttattaggggtgttaatcagcacaaatgagcaactggctcatcagtcggtgcaggctgacaggtgcaggaaatacggagggcaggcggggtagggggcacggaatgcttcccaacatgagggcatctcaggccagcaggcggggcccagagacccagaagcaccacaactcccccgtgtccacaaggcactttatgcattcaaaaccaccgaattcacacccaggtttgctcagacagaggcccagaggcgaccccgctctggcgtggctaccacctgagcggctggcggccctggcccagctcggcctccgcgtaggcgtcatacagcaccttcaggtgcaacagcagctgctccaggttctcgccggtcaacgccgacagcacgatgacctcctgtcccaagtgatcccggagctgggacagattggcttgggcttcagggaggtcaatcttgtttgcgacgattgcgtggggcctcgcagacaggcccttttcatacatctccagttcatattttaaatcgtcaacttgagtccacggctcaggctgagaaagatccaccacgaacaagagaaagcggcagcgctcgatgtgcctgaggaaggcggaccccagacccctgttctggtgggcgcctcgtatgatgccggggatgtcggccactgctatttgtaggtggccttcgtagtggacgatcccgacgtggggcttcagggtggtgaacgggtaggaagccacggcgggtctggcgtttgaaatggcccggagcagtgaggacttcccggcgttggggaatcccaccattccggcgtgggccaccgtcttgagctccaggtggagaactcgctgctgtcctggctgtccaggggtacaggtcacaggggcacggttgttgttggccaggaagaagcggttgcctttccctcctgccccgcccagcgcggcaatgtactcatctcccacgcaagacaggtcggccacaactctgcctccctccttcaccagcgtgcccacggggacccggatgtagaggacggcgccactgcgcccgaagcagtttttactccctccatcttctccactgaaaccctggtaccgcgacaggaccgacgacagggacttgacttgctggtcaactctcagaatgacgtgtccaccgttgcctccgtcccctccatcagggcctccaaactccttgcggggctcactgtggaagcagcttgccccagcgcctccgtttcctccacagacaagcactctccgatagtccacaaagtaccttttcagctttttctcagagagcagcttcttccccgggagttcctgatgcttggcgaggtccgcacggccgaccgagagcagcctgggagaagcccgctgtggcagtagccggctgggcttcaggccagcccatgtggacaaagcccaatgccccacgccctgaaacacggtcctcaatcttgctgagaaacaccttgcaggtgccatggcccctcacgtcaaaaatatctggaa

SEQ ID NO: 10939 - RNA, 2880 nt, Homo sapiens
  source 1..2880: mol_type = other RNA
ctgaatagctgggactacaggtgaccgccaccacgcctggctaatttttttgtatttttagtagagacggggtttcactgtgttagccaggatggtctcaatctcctgaccttgtgatccaccagcctcggcctcccaaagtgctgggactacaggcatgagccaccgtgcccagaatgttctgtttttgtttgtttgtttgtttgttttttgagacagggtctcgctctgtcactcaggctggagtgcagtggtgcaatcacggctcactgcagccttgacctcccaggctcacatgatcctcccacgacagcctctggagtgtcccctccactttctttcttaggggcccctcagggacatgtcagaggcctgagactacttgggggatgtctatgggccaggcaggctgccagcagctgagctgtccttgccctggggctcctctgcagtcagggagacaccaggcatgggcctggcttggatgcatcagtacttgactgcaaagacttaaaccacagacaggaaaggcgctgctgcagtctcgacggtcaaatgcagggccccctcagctgccatcccactgaggggcgaaggcccatcatctcccttcggctcggtaactgcctggcgtagcacaagggttctctttaaatccccagcaaatggagctgagtggaaattccgccccatattaccaggcacacgtctccttccactcctcactataccctgcccatgccacggccgccttctgagaataacgctgacagttccatggcccacagcccctctagttaacttgctgtgcacacggcagcccagccagaaacacgcagccaggtcggatattgggtgcattcagtcgtgaagcctgaggcttcctggctcccactgagcacagagaagtgttctgaaggacaggaagcagctggcctcactgctcttctcagacggctgatggagaaaagctcacagctgcctgcgccgctctgcctggacttgcatcctcggccccaccccttgcgcagcagtgaggccccccgagacactggtgcctgggcttgcggtaccgcagggctgctggacaacgggccagacgcagccccagtgtggatccagaggtctctctccgtagcaagccatggaagcacgacgggcactgtgctgagaaccctggtctgcacttctgacctggggctctggctgtgcggttctgctgagctcatccgagagtccacgcgtgcatggcggagacctgagtcagcggcagggccaccccgttatgggcaccccaaccccttattaggggtgttaatcagcacaaatgagcaactggctcatcagtcggtgcaggctgacaggtgcaggaaatacggagggcaggcggggtagggggcacggaatgcttcccaacatgagggcatctcaggccagcaggcggggcccagagacccagaagcaccacaactcccccgtgtccacaaggcactttatgcattcaaaaccaccgaattcacacccaggtttgctcagacagaggcccagaggcgaccccgctctggcgtggctaccacctgagcggctggcggccctggcccagctcggcctccgcgtaggcgtcatacagcaccttcaggtgcaacagcagctgctccaggttctcgccggtcaacgccgacagcacgatgacctcctgtcccaagtgatcccggagctgggacagattggcttgggcttcagggaggtcaatcttgtttgcgacgattgcgtggggcctcgcagacaggcccttttcatacatctccagttcatattttaaatcgtcaacttgagtccacggctcaggctgagaaagatccaccacgaacaagagaaagcggcagcgctcgatgtgcctgaggaaggcggaccccagacccctgttctggtgggcgcctcgtatgatgccggggatgtcggccactgctatttgtaggtggccttcgtagtggacgatcccgacgtggggcttcagggtggtgaacgggtaggaagccacggcgggtctggcgtttgaaatggcccggagcagtgaggacttcccggcgttggggaatcccaccattccggcgtgggccaccgtcttgagctccaggtggagaactcgctgctgtcctggctgtccaggggtacaggtcacaggggcacggttgttgttggccaggaagaagcggttgcctttccctcctgccccgcccagcgcggcaatgtactcatctcccacgcaagacaggtcggccacaactctgcctccctccttcaccagcgtgcccacggggacccggatgtagaggacggcgccactgcgcccgaagcagtttttactccctccatcttctccactgaaaccctggtaccgcgacaggaccgacgacagggacttgacttgctggtcaactctcagaatgacgtgtccaccgttgcctccgtcccctccatcagggcctccaaactccttgcggggctcactgtggaagcagcttgccccagcgcctccgtttcctccacagacaagcactctccgatagtccacaaagtaccttttcctgtgccttctgaggaggagacaggcaagctgctctaactccaggagtctcaccagctttttctcagagagcagcttcttccccgggagttcctgatgcttggcgaggtccgcacggccgaccgagagcagcctgggagaagcccgctgtggcagtagccggctgggcttcaggccagcccatgtggacaaagcccaatgccccacgccctgaaacacggtcctcaatcttgctgagaaacaccttgcaggtgccatggccccggctcgggaaagcacgtcacttccggagc

SEQ ID NO: 10940 - RNA, 2617 nt, Homo sapiens
  source 1..2617: mol_type = other RNA
ctgaatagctgggactacaggtgaccgccaccacgcctggctaatttttttgtatttttagtagagacggggtttcactgtgttagccaggatggtctcaatctcctgaccttgtgatccaccagcctcggcctcccaaagtgctgggactacaggcatgagccaccgtgcccagaatgttctgtttttgtttgtttgtttgtttgttttttgagacagggtctcgctctgtcactcaggctggagtgcagtggtgcaatcacggctcactgcagccttgacctcccaggctcacatgatcctcccacgacagcctctggagtgtcccctccactttctttcttaggggcccctcagggacatgtcagaggcctgagactacttgggggatgtctatgggccaggcaggctgccagcagctgagctgtccttgccctggggctcctctgcagtcagggagacaccaggcatgggcctggcttggatgcatcagtacttgactgcaaagacttaaaccacagacaggaaaggcgctgctgcagtctcgacggtcaaatgcagggccccctcagctgccatcccactgaggggcgaaggcccatcatctcccttcggctcggtaactgcctggcgtagcacaagggttctctttaaatccccagcaaatggagctgagtggaaattccgccccatattaccaggcacacgtctccttccactcctcactataccctgcccatgccacggccgccttctgagaataacgctgacagttccatggcccacagcccctctagttaacttgctgtgcacacggcagcccagccagaaacacgcagccaggtcggatattgggtgcattcagtcgtgaagcctgaggcttcctggctcccactgagcacagagaagtgttctgaaggacaggaagcagctggcctcactgctcttctcagacggctgatggagaaaagctcacagctgcctgcgccgctctgcctggacttgcatcctcggccccaccccttgcgcagcagtgaggccccccgagacactggtgcctgggcttgcggtaccgcagggctgctggacaacgggccagacgcagccccagtgtggatccagaggtctctctccgtagcaagccatggaagcacgacgggcactgtgctgagaaccctggtctgcacttctgacctggggctctggctgtgcggttctgctgagctcatccgagagtccacgcgtgcatggcggagacctgagtcagcggcagggccaccccgttatgggcaccccaaccccttattaggggtgttaatcagcacaaatgagcaactggctcatcagtcggtgcaggctgacaggtgcaggaaatacggagggcaggcggggtagggggcacggaatgcttcccaacatgagggcatctcaggccagcaggcggggcccagagacccagaagcaccacaactcccccgtgtccacaaggcactttatgcattcaaaaccaccgaattcacacccaggtttgctcagacagaggcccagaggcgaccccgctctggcgtggctaccacctgagcggctggcggccctggcccagctcggcctccgcgtaggcgtcatacagcaccttcaggtgcaacagcagctgctccaggttctcgccggtcaacgccgacagcacgatgacctcctgtcccaagtgatcccggagctgggacagattggcttgggcttcagggaggtcaatcttgtttgcgacgattgcgtggggcctcgcagacaggcccttttcatacatctccagttcatattttaaatcgtcaacttgagtccacggctcaggctgagaaagatccaccacgaacaagagaaagcggcagcgctcgatgtgcctgaggaaggcggaccccagacccctgttctggtgggcgcctcgtatgatgccggggatgtcggccactgctatttgtaggtggccttcgtagtggacgatcccgacgtggggcttcagggtggtgaacgggtaggaagccacggcgggtctggcgtttgaaatggcccggagcagtgaggacttcccggcgttggggaatcccaccattccggcgtgggccaccgtcttgagctccaggtggagaactcgctgctgtcctggctgtccaggggtacaggtcacaggggcacggttgttgttggccaggaagaagcggttgcctttccctcctgccccgcccagcgcggcaatgtactcatctcccacgcaagacaggtcggccacaactctgcctccctccttcaccagcgtgcccacggggacccggatgtagaggacggcgccactgcgcccgaagcagtttttactccctccatcttctccactgaaaccctggtaccgcgacaggaccgacgacagggacttgacttgctggtcaactctcagaatgacgtgtccaccgttgcctccgtcccctccatcagggcctccaaactccttgcggggctcactgtggaagcagcttgccccagcgcctccgtttcctccacagacaagcactctccgatagtccacaaagtaccttttcggctcgggaaagcacgtcacttccggagc

SEQ ID NO: 10941 - RNA, 2963 nt, Homo sapiens
  source 1..2963: mol_type = other RNA
ctgaatagctgggactacaggtgaccgccaccacgcctggctaatttttttgtatttttagtagagacggggtttcactgtgttagccaggatggtctcaatctcctgaccttgtgatccaccagcctcggcctcccaaagtgctgggactacaggcatgagccaccgtgcccagaatgttctgtttttgtttgtttgtttgtttgttttttgagacagggtctcgctctgtcactcaggctggagtgcagtggtgcaatcacggctcactgcagccttgacctcccaggctcacatgatcctcccacgacagcctctggagtgtcccctccactttctttcttaggggcccctcagggacatgtcagaggcctgagactacttgggggatgtctatgggccaggcaggctgccagcagctgagctgtccttgccctggggctcctctgcagtcagggagacaccaggcatgggcctggcttggatgcatcagtacttgactgcaaagacttaaaccacagacaggaaaggcgctgctgcagtctcgacggtcaaatgcagggccccctcagctgccatcccactgaggggcgaaggcccatcatctcccttcggctcggtaactgcctggcgtagcacaagggttctctttaaatccccagcaaatggagctgagtggaaattccgccccatattaccaggcacacgtctccttccactcctcactataccctgcccatgccacggccgccttctgagaataacgctgacagttccatggcccacagcccctctagttaacttgctgtgcacacggcagcccagccagaaacacgcagccaggtcggatattgggtgcattcagtcgtgaagcctgaggcttcctggctcccactgagcacagagaagtgttctgaaggacaggaagcagctggcctcactgctcttctcagacggctgatggagaaaagctcacagctgcctgcgccgctctgcctggacttgcatcctcggccccaccccttgcgcagcagtgaggccccccgagacactggtgcctgggcttgcggtaccgcagggctgctggacaacgggccagacgcagccccagtgtggatccagaggtctctctccgtagcaagccatggaagcacgacgggcactgtgctgagaaccctggtctgcacttctgacctggggctctggctgtgcggttctgctgagctcatccgagagtccacgcgtgcatggcggagacctgagtcagcggcagggccaccccgttatgggcaccccaaccccttattaggggtgttaatcagcacaaatgagcaactggctcatcagtcggtgcaggctgacaggtgcaggaaatacggagggcaggcggggtagggggcacggaatgcttcccaacatgagggcatctcaggccagcaggcggggcccagagacccagaagcaccacaactcccccgtgtccacaaggcactttatgcattcaaaaccaccgaattcacacccaggtttgctcagacagaggcccagaggcgaccccgctctggcgtggctaccacctgagcggctggcggccctggcccagctcggcctccgcgtaggcgtcatacagcaccttcaggtgcaacagcagctgctccaggttctcgccggtcaacgccgacagcacgatgacctcctgtcccaagtgatcccggagctgggacagattggcttgggcttcagggaggtcaatcttgtttgcgacgattgcgtggggcctcgcagacaggcccttttcatacatctccagttcatattttaaatcgtcaacttgagtccacggctcaggctgagaaagatccaccacgaacaagagaaagcggcagcgctcgatgtgcctgaggaaggcggaccccagacccctgttctggtgggcgcctcgtatgatgccggggatgtcggccactgctatttgtaggtggccttcgtagtggacgatcccgacgtggggcttcagggtggtgaacgggtaggaagccacggcgggtctggcgtttgaaatggcccggagcagtgaggacttcccggcgttggggaatcccaccattccggcgtgggccaccgtcttgagctccaggtggagaactcgctgctgtcctggctgtccaggggtacaggtcacaggggcacggttgttgttggccaggaagaagcggttgcctttccctcctgccccgcccagcgcggcaatgtactcatctcccacgcaagacaggtcggccacaactctgcctccctccttcaccagcgtgcccacggggacccggatgtagaggacggcgccactgcgcccgaagcagtttttactccctccatcttctccactgaaaccctggtaccgcgacaggaccgacgacagggacttgacttgctggtcaactctcagaatgacgtgtccaccgttgcctccgtcccctccatcagggcctccaaactccttgcggggctcactgtggaagcagcttgccccagcgcctccgtttcctccacagacaagcactctccgatagtccacaaagtaccttttcgtgttggccaggatggtctcgatctcctgacctcgtgatccacccgcctcggcctcccaaagtgctgggactacaggcgtgagccactgtgcccggctaggaaagctgttctgtaggtcactaaggtaggtgcaatcagctttttctcagagagcagcttcttccccgggagttcctgatgcttggcgaggtccgcacggccgaccgagagcagcctgggagaagcccgctgtggcagtagccggctgggcttcaggccagcccatgtggacaaagcccaatgccccacgccctgaaacacggtcctcaatcttgctgagaaacaccttgcaggtgccatggccccggctcgggaaagcacgtcacttccggagc

SEQ ID NO: 10942 - RNA, 2822 nt, Homo sapiens
  source 1..2822: mol_type = other RNA
ctgaatagctgggactacaggtgaccgccaccacgcctggctaatttttttgtatttttagtagagacggggtttcactgtgttagccaggatggtctcaatctcctgaccttgtgatccaccagcctcggcctcccaaagtgctgggactacaggcatgagccaccgtgcccagaatgttctgtttttgtttgtttgtttgtttgttttttgagacagggtctcgctctgtcactcaggctggagtgcagtggtgcaatcacggctcactgcagccttgacctcccaggctcacatgatcctcccacgacagcctctggagtgtcccctccactttctttcttaggggcccctcagggacatgtcagaggcctgagactacttgggggatgtctatgggccaggcaggctgccagcagctgagctgtccttgccctggggctcctctgcagtcagggagacaccaggcatgggcctggcttggatgcatcagtacttgactgcaaagacttaaaccacagacaggaaaggcgctgctgcagtctcgacggtcaaatgcagggccccctcagctgccatcccactgaggggcgaaggcccatcatctcccttcggctcggtaactgcctggcgtagcacaagggttctctttaaatccccagcaaatggagctgagtggaaattccgccccatattaccaggcacacgtctccttccactcctcactataccctgcccatgccacggccgccttctgagaataacgctgacagttccatggcccacagcccctctagttaacttgctgtgcacacggcagcccagccagaaacacgcagccaggtcggatattgggtgcattcagtcgtgaagcctgaggcttcctggctcccactgagcacagagaagtgttctgaaggacaggaagcagctggcctcactgctcttctcagacggctgatggagaaaagctcacagctgcctgcgccgctctgcctggacttgcatcctcggccccaccccttgcgcagcagtgaggccccccgagacactggtgcctgggcttgcggtaccgcagggctgctggacaacgggccagacgcagccccagtgtggatccagaggtctctctccgtagcaagccatggaagcacgacgggcactgtgctgagaaccctggtctgcacttctgacctggggctctggctgtgcggttctgctgagctcatccgagagtccacgcgtgcatggcggagacctgagtcagcggcagggccaccccgttatgggcaccccaaccccttattaggggtgttaatcagcacaaatgagcaactggctcatcagtcggtgcaggctgacaggtgcaggaaatacggagggcaggcggggtagggggcacggaatgcttcccaacatgagggcatctcaggccagcaggcggggcccagagacccagaagcaccacaactcccccgtgtccacaaggcactttatgcattcaaaaccaccgaattcacacccaggtttgctcagacagaggcccagaggcgaccccgctctggcgtggctaccacctgagcggctggcggccctggcccagctcggcctccgcgtaggcgtcatacagcaccttcaggtgcaacagcagctgctccaggttctcgccggtcaacgccgacagcacgatgacctcctgtcccaagtgatcccggagctgggacagattggcttgggcttcagggaggtcaatcttgtttgcgacgattgcgtggggcctcgcagacaggcccttttcatacatctccagttcatattttaaatcgtcaacttgagtccacggctcaggctgagaaagatccaccacgaacaagagaaagcggcagcgctcgatgtgcctgaggaaggcggaccccagacccctgttctggtgggcgcctcgtatgatgccggggatgtcggccactgctatttgtaggtggccttcgtagtggacgatcccgacgtggggcttcagggtggtgaacgggtaggaagccacggcgggtctggcgtttgaaatggcccggagcagtgaggacttcccggcgttggggaatcccaccattccggcgtgggccaccgtcttgagctccaggtggagaactcgctgctgtcctggctgtccaggggtacaggtcacaggggcacggttgttgttggccaggaagaagcggttgcctttccctcctgccccgcccagcgcggcaatgtactcatctcccacgcaagacaggtcggccacaactctgcctccctccttcaccagcgtgcccacggggacccggatgtagaggacggcgccactgcgcccgaagcagtttttactccctccatcttctccactgaaaccctggtaccgcgacaggaccgacgacagggacttgacttgctggtcaactctcagaatgacgtgtccaccgttgcctccgtcccctccatcagggcctccaaactccttgcggggctcactgtggaagcagcttgccccagcgcctccgtttcctccacagacaagcactctccgatagtccacaaagtacctttttttttctcagagagcagcttcttccccgggagttcctgatgcttggcgaggtccgcacggccgaccgagagcagcctgggagaagcccgctgtggcagtagccggctgggcttcaggccagcccatgtggacaaagcccaatgccccacgccctgaaacacggtcctcaatcttgctgagaaacaccttgcaggtgccatggccccggctcgggaaagcacgtcacttccggagc

SEQ ID NO: 10943 - RNA, 2830 nt, Homo sapiens
  source 1..2830: mol_type = other RNA
ctgaatagctgggactacaggtgaccgccaccacgcctggctaatttttttgtatttttagtagagacggggtttcactgtgttagccaggatggtctcaatctcctgaccttgtgatccaccagcctcggcctcccaaagtgctgggactacaggcatgagccaccgtgcccagaatgttctgtttttgtttgtttgtttgtttgttttttgagacagggtctcgctctgtcactcaggctggagtgcagtggtgcaatcacggctcactgcagccttgacctcccaggctcacatgatcctcccacgacagcctctggagtgtcccctccactttctttcttaggggcccctcagggacatgtcagaggcctgagactacttgggggatgtctatgggccaggcaggctgccagcagctgagctgtccttgccctggggctcctctgcagtcagggagacaccaggcatgggcctggcttggatgcatcagtacttgactgcaaagacttaaaccacagacaggaaaggcgctgctgcagtctcgacggtcaaatgcagggccccctcagctgccatcccactgaggggcgaaggcccatcatctcccttcggctcggtaactgcctggcgtagcacaagggttctctttaaatccccagcaaatggagctgagtggaaattccgccccatattaccaggcacacgtctccttccactcctcactataccctgcccatgccacggccgccttctgagaataacgctgacagttccatggcccacagcccctctagttaacttgctgtgcacacggcagcccagccagaaacacgcagccaggtcggatattgggtgcattcagtcgtgaagcctgaggcttcctggctcccactgagcacagagaagtgttctgaaggacaggaagcagctggcctcactgctcttctcagacggctgatggagaaaagctcacagctgcctgcgccgctctgcctggacttgcatcctcggccccaccccttgcgcagcagtgaggccccccgagacactggtgcctgggcttgcggtaccgcagggctgctggacaacgggccagacgcagccccagtgtggatccagaggtctctctccgtagcaagccatggaagcacgacgggcactgtgctgagaaccctggtctgcacttctgacctggggctctggctgtgcggttctgctgagctcatccgagagtccacgcgtgcatggcggagacctgagtcagcggcagggccaccccgttatgggcaccccaaccccttattaggggtgttaatcagcacaaatgagcaactggctcatcagtcggtgcaggctgacaggtgcaggaaatacggagggcaggcggggtagggggcacggaatgcttcccaacatgagggcatctcaggccagcaggcggggcccagagacccagaagcaccacaactcccccgtgtccacaaggcactttatgcattcaaaaccaccgaattcacacccaggtttgctcagacagaggcccagaggcgaccccgctctggcgtggctaccacctgagcggctggcggccctggcccagctcggcctccgcgtaggcgtcatacagcaccttcaggtgcaacagcagctgctccaggttctcgccggtcaacgccgacagcacgatgacctcctgtcccaagtgatcccggagctgggacagattggcttgggcttcagggaggtcaatcttgtttgcgacgattgcgtggggcctcgcagacaggcccttttcatacatctccagttcatattttaaatcgtcaacttgagtccacggctcaggctgagaaagatccaccacgaacaagagaaagcggcagcgctcgatgtgcctgaggaaggcggaccccagacccctgttctggtgggcgcctcgtatgatgccggggatgtcggccactgctatttgtaggtggccttcgtagtggacgatcccgacgtggggcttcagggtggtgaacgggtaggaagccacggcgggtctggcgtttgaaatggcccggagcagtgaggacttcccggcgttggggaatcccaccattccggcgtgggccaccgtcttgagctccaggtggagaactcgctgctgtcctggctgtccaggggtacaggtcacaggggcacggttgttgttggccaggaagaagcggttgcctttccctcctgccccgcccagcgcggcaatgtactcatctcccacgcaagacaggtcggccacaactctgcctccctccttcaccagcgtgcccacggggacccggatgtagaggacggcgccactgcgcccgaagcagtttttactccctccatcttctccactgaaaccctggtaccgcgacaggaccgacgacagggacttgacttgctggtcaactgcctctcagaatgacgtgtccaccgttgcctccgtcccctccatcagggcctccaaactccttgcggggctcactgtggaagcagcttgccccagcgcctccgtttcctccacagacaagcactctccgatagtccacaaagtaccttttcagctttttctcagagagcagcttcttccccgggagttcctgatgcttggcgaggtccgcacggccgaccgagagcagcctgggagaagcccgctgtggcagtagccggctgggcttcaggccagcccatgtggacaaagcccaatgccccacgccctgaaacacggtcctcaatcttgctgagaaacaccttgcaggtgccatggccccggctcgggaaagcacgtcacttccggagc

SEQ ID NO: 10944 - RNA, 2353 nt, Homo sapiens
  source 1..2353: mol_type = other RNA
ctgaatagctgggactacaggtgaccgccaccacgcctggctaatttttttgtatttttagtagagacggggtttcactgtgttagccaggatggtctcaatctcctgaccttgtgatccaccagcctcggcctcccaaagtgctgggactacaggcatgagccaccgtgcccagaatgttctgtttttgtttgtttgtttgtttgttttttgagacagggtctcgctctgtcactcaggctggagtgcagtggtgcaatcacggctcactgcagccttgacctcccaggctcacatgatcctcccacgacagcctctggagtgtcccctccactttctttcttaggggcccctcagggacatgtcagaggcctgagactacttgggggatgtctatgggccaggcaggctgccagcagctgagctgtccttgccctggggctcctctgcagtcagggagacaccaggcatgggcctggcttggatgcatcagtacttgactgcaaagacttaaaccacagacaggaaaggcgctgctgcagtctcgacggtcaaatgcagggccccctcagctgccatcccactgaggggcgaaggcccatcatctcccttcggctcggtaactgcctggcgtagcacaagggttctctttaaatccccagcaaatggagctgagtggaaattccgccccatattaccaggcacacgtctccttccactcctcactataccctgcccatgccacggccgccttctgagaataacgctgacagttccatggcccacagcccctctagttaacttgctgtgcacacggcagcccagccagaaacacgcagccaggtcggatattgggtgcattcagtcgtgaagcctgaggcttcctggctcccactgagcacagagaagtgttctgaaggacaggaagcagctggcctcactgctcttctcagacggctgatggagaaaagctcacagctgcctgcgccgctctgcctggacttgcatcctcggccccaccccttgcgcagcagtgaggccccccgagacactggtgcctgggcttgcggtaccgcagggctgctggacaacgggccagacgcagccccagtgtggatccagaggtctctctccgtagcaagccatggaagcacgacgggcactgtgctgagaaccctggtctgcacttctgacctggggctctggctgtgcggttctgctgagctcatccgagagtccacgcgtgcatggcggagacctgagtcagcggcagggccaccccgttatgggcaccccaaccccttattaggggtgttaatcagcacaaatgagcaactggctcatcagtcggtgcaggctgacaggtgcaggaaatacggagggcaggcggggtagggggcacggaatgcttcccaacatgagggcatctcaggccagcaggcggggcccagagacccagaagcaccacaactcccccgtgtccacaaggcactttatgcattcaaaaccaccgaattcacacccaggtttgctcagacagaggcccagaggcgaccccgctctggcgtggctaccacctgagcggctggcggccctggcccagctcggcctccgcgtaggcgtcatacagcaccttcaggtgcaacagcagctgctccaggttctcgccggtcaacgccgacagcacgatgacctcctgtcccaagtgatcccggagctgggacagattggcttgggcttcagggaggtcaatcttgtttgcgacgattgcgtggggcctcgcagacaggcccttttcatacatctccagttcatattttaaatcgtcaacttgagtccacggctcaggctgagaaagatccaccacgaacaagagaaagcggcagcgctcgatgtgcctgaggaaggcggaccccagacccctgttctggtgggcgcctcgtatgatgccggggatgtcggccactgctatttgtaggtggccttcgtagtggacgatcccgacgtggggcttcagggtggtgaacgggtaggaagccacggcgggtctggcgtttgaaatggcccggagcagtgaggacttcccggcgttggggaatcccaccattccggcgtgggccaccgtcttgagctccaggtggagaactcgctgctgtcctggctgtccaggggtacaggtcacaggggcacggttgttgttggccaggaagaagcggttgcctttccctcctgccccgcccagcgcggcaatgtactcatctcccacgcaagacaggtcggccacaactctgcctccctccttcaccagcgtgcccacggggaccggctcgggaaagcacgtcacttccggagc

SEQ ID NO: 10945 - RNA, 2918 nt, Homo sapiens
  source 1..2918: mol_type = other RNA
ctgaatagctgggactacaggtgaccgccaccacgcctggctaatttttttgtatttttagtagagacggggtttcactgtgttagccaggatggtctcaatctcctgaccttgtgatccaccagcctcggcctcccaaagtgctgggactacaggcatgagccaccgtgcccagaatgttctgtttttgtttgtttgtttgtttgttttttgagacagggtctcgctctgtcactcaggctggagtgcagtggtgcaatcacggctcactgcagccttgacctcccaggctcacatgatcctcccacgacagcctctggagtgtcccctccactttctttcttaggggcccctcagggacatgtcagaggcctgagactacttgggggatgtctatgggccaggcaggctgccagcagctgagctgtccttgccctggggctcctctgcagtcagggagacaccaggcatgggcctggcttggatgcatcagtacttgactgcaaagacttaaaccacagacaggaaaggcgctgctgcagtctcgacggtcaaatgcagggccccctcagctgccatcccactgaggggcgaaggcccatcatctcccttcggctcggtaactgcctggcgtagcacaagggttctctttaaatccccagcaaatggagctgagtggaaattccgccccatattaccaggcacacgtctccttccactcctcactataccctgcccatgccacggccgccttctgagaataacgctgacagttccatggcccacagcccctctagttaacttgctgtgcacacggcagcccagccagaaacacgcagccaggtcggatattgggtgcattcagtcgtgaagcctgaggcttcctggctcccactgagcacagagaagtgttctgaaggacaggaagcagctggcctcactgctcttctcagacggctgatggagaaaagctcacagctgcctgcgccgctctgcctggacttgcatcctcggccccaccccttgcgcagcagtgaggccccccgagacactggtgcctgggcttgcggtaccgcagggctgctggacaacgggccagacgcagccccagtgtggatccagaggtctctctccgtagcaagccatggaagcacgacgggcactgtgctgagaaccctggtctgcacttctgacctggggctctggctgtgcggttctgctgagctcatccgagagtccacgcgtgcatggcggagacctgagtcagcggcagggccaccccgttatgggcaccccaaccccttattaggggtgttaatcagcacaaatgagcaactggctcatcagtcggtgcaggctgacaggtgcaggaaatacggagggcaggcggggtagggggcacggaatgcttcccaacatgagggcatctcaggccagcaggcggggcccagagacccagaagcaccacaactcccccgtgtccacaaggcactttatgcattcaaaaccaccgaattcacacccaggtttgctcagacagaggcccagaggcgaccccgctctggcgtggctaccacctgagcggctggcggccctggcccagctcggcctccgcgtaggcgtcatacagcaccttcaggtgcaacagcagctgctccaggttctcgccggtcaacgccgacagcacgatgacctcctgtcccaagtgatcccggagctgggacagattggcttgggcttcagggaggtcaatcttgtttgcgacgattgcgtggggcctcgcagacaggcccttttcatacatctccagttcatattttaaatcgtcaacttgagtccacggctcaggctgagaaagatccaccacgaacaagagaaagcggcagcgctcgatgtgcctgaggaaggcggaccccagacccctgttctggtgggcgcctcgtatgatgccggggatgtcggccactttgggagaattctggaagttctacctgctatttgtaggtggccttcgtagtggacgatcccgacgtggggcttcagggtggtgaacgggtaggaagccacggcgggtctggcgtttgaaatggcccggagcagtgaggacttcccggcgttggggaatcccaccattccggcgtgggccaccgtcttgagctccaggtggagaactcgctgctgtcctggctgtccaggggtacaggtcacaggggcacggttgttgttggccaggaagaagcggttgcctttccctcctgccccgcccagcgcggcaatgtactcatctcccacgcaagacaggtcggccacaactctgcctccctccttcaccagcgtgcccacggggacccggatgtagaggacggcgccactgcgcccgaagcagtttttactccctccatcttctccactgaaaccctggtaccgcgacaggaccgacgacagggacttgacttgctggtcaacacacaggcctcgtgctttcacgcgaccgacatgtcagcttccctgacaggaaactctctgtgctcctctcagaatgacgtgtccaccgttgcctccgtcccctccatcagggcctccaaactccttgcggggctcactgtggaagcagcttgccccagcgcctccgtttcctccacagacaagcactctccgatagtccacaaagtaccttttcagctttttctcagagagcagcttcttccccgggagttcctgatgcttggcgaggtccgcacggccgaccgagagcagcctgggagaagcccgctgtggcagtagccggctgggcttcaggccagcccatgtggacaaagcccaatgccccacgccctgaaacacggtcctcaatcttgctgagaaacaccttgcaggtgccatggccccggctcgggaaagcacgtcacttccggagc

SEQ ID NO: 10946 - RNA, 2709 nt, Homo sapiens
  source 1..2709: mol_type = other RNA
ctgaatagctgggactacaggtgaccgccaccacgcctggctaatttttttgtatttttagtagagacggggtttcactgtgttagccaggatggtctcaatctcctgaccttgtgatccaccagcctcggcctcccaaagtgctgggactacaggcatgagccaccgtgcccagaatgttctgtttttgtttgtttgtttgtttgttttttgagacagggtctcgctctgtcactcaggctggagtgcagtggtgcaatcacggctcactgcagccttgacctcccaggctcacatgatcctcccacgacagcctctggagtgtcccctccactttctttcttaggggcccctcagggacatgtcagaggcctgagactacttgggggatgtctatgggccaggcaggctgccagcagctgagctgtccttgccctggggctcctctgcagtcagggagacaccaggcatgggcctggcttggatgcatcagtacttgactgcaaagacttaaaccacagacaggaaaggcgctgctgcagtctcgacggtcaaatgcagggccccctcagctgccatcccactgaggggcgaaggcccatcatctcccttcggctcggtaactgcctggcgtagcacaagggttctctttaaatccccagcaaatggagctgagtggaaattccgccccatattaccaggcacacgtctccttccactcctcactataccctgcccatgccacggccgccttctgagaataacgctgacagttccatggcccacagcccctctagttaacttgctgtgcacacggcagcccagccagaaacacgcagccaggtcggatattgggtgcattcagtcgtgaagcctgaggcttcctggctcccactgagcacagagaagtgttctgaaggacaggaagcagctggcctcactgctcttctcagacggctgatggagaaaagctcacagctgcctgcgccgctctgcctggacttgcatcctcggccccaccccttgcgcagcagtgaggccccccgagacactggtgcctgggcttgcggtaccgcagggctgctggacaacgggccagacgcagccccagtgtggatccagaggtctctctccgtagcaagccatggaagcacgacgggcactgtgctgagaaccctggtctgcacttctgacctggggctctggctgtgcggttctgctgagctcatccgagagtccacgcgtgcatggcggagacctgagtcagcggcagggccaccccgttatgggcaccccaaccccttattaggggtgttaatcagcacaaatgagcaactggctcatcagtcggtgcaggctgacaggtgcaggaaatacggagggcaggcggggtagggggcacggaatgcttcccaacatgagggcatctcaggccagcaggcggggcccagagacccagaagcaccacaactcccccgtgtccacaaggcactttatgcattcaaaaccaccgaattcacacccaggtttgctcagacagaggcccagaggcgaccccgctctggcgtggctaccacctgagcggctggcggccctggcccagctcggcctccgcgtaggcgtcatacagcaccttcaggtgcaacagcagctgctccaggttctcgccggtcaacgccgacagcacgatgacctcctgtcccaagtgatcccggagctgggacagattggcttgggcttcagggaggtcaatcttgtttgcgacgattgcgtggggcctcgcagacaggcccttttcatacatctccagttcatattttaaatcgtcaacttgagtccacggctcaggctgagaaagatccaccacgaacaagagaaagcggcagcgctcgatgtgcctgaggaaggcggaccccagacccctgttctggtgggcgcctcgtatgatgccggggatgtcggccactttgggagaattctggaagttctacctgctatttgtaggtggccttcgtagtggacgatcccgacgtggggcttcagggtggtgaacgggtaggaagccacggcgggtctggcgtttgaaatggcccggagcagtgaggacttcccggcgttggggaatcccaccattccggcgtgggccaccgtcttgagctccaggtggagaactcgctgctgtcctggctgtccaggggtacaggtcacaggggcacggttgttgttggccaggaagaagcggttgcctttccctcctgccccgcccagcgcggcaatgtactcatctcccacgcaagacaggtcggccacaactctgcctccctccttcaccagcgtgcccacggggacccggatgtagaggacggcgccactgcgcccgaagcagtttttactccctccatcttctccactgaaaccctggtaccgcgacaggaccgacgacagggacttgacttgctggtcaacacacaggcctcgtgctttcacgcgaccgacatgtcagcttccctgacaggaaactctctgtgctcctctcagaatgacgtgtccaccgttgcctccgtcccctccatcagggcctccaaactccttgcggggctcactgtggaagcagcttgccccagcgcctccgtttcctccacagacaagcactctccgatagtccacaaagtaccttttcggctcgggaaagcacgtcacttccggagc

SEQ ID NO: 10947 - RNA, 2845 nt, Homo sapiens
  source 1..2845: mol_type = other RNA
ctgaatagctgggactacaggtgaccgccaccacgcctggctaatttttttgtatttttagtagagacggggtttcactgtgttagccaggatggtctcaatctcctgaccttgtgatccaccagcctcggcctcccaaagtgctgggactacaggcatgagccaccgtgcccagaatgttctgtttttgtttgtttgtttgtttgttttttgagacagggtctcgctctgtcactcaggctggagtgcagtggtgcaatcacggctcactgcagccttgacctcccaggctcacatgatcctcccacgacagcctctggagtgtcccctccactttctttcttaggggcccctcagggacatgtcagaggcctgagactacttgggggatgtctatgggccaggcaggctgccagcagctgagctgtccttgccctggggctcctctgcagtcagggagacaccaggcatgggcctggcttggatgcatcagtacttgactgcaaagacttaaaccacagacaggaaaggcgctgctgcagtctcgacggtcaaatgcagggccccctcagctgccatcccactgaggggcgaaggcccatcatctcccttcggctcggtaactgcctggcgtagcacaagggttctctttaaatccccagcaaatggagctgagtggaaattccgccccatattaccaggcacacgtctccttccactcctcactataccctgcccatgccacggccgccttctgagaataacgctgacagttccatggcccacagcccctctagttaacttgctgtgcacacggcagcccagccagaaacacgcagccaggtcggatattgggtgcattcagtcgtgaagcctgaggcttcctggctcccactgagcacagagaagtgttctgaaggacaggaagcagctggcctcactgctcttctcagacggctgatggagaaaagctcacagctgcctgcgccgctctgcctggacttgcatcctcggccccaccccttgcgcagcagtgaggccccccgagacactggtgcctgggcttgcggtaccgcagggctgctggacaacgggccagacgcagccccagtgtggatccagaggtctctctccgtagcaagccatggaagcacgacgggcactgtgctgagaaccctggtctgcacttctgacctggggctctggctgtgcggttctgctgagctcatccgagagtccacgcgtgcatggcggagacctgagtcagcggcagggccaccccgttatgggcaccccaaccccttattaggggtgttaatcagcacaaatgagcaactggctcatcagtcggtgcaggctgacaggtgcaggaaatacggagggcaggcggggtagggggcacggaatgcttcccaacatgagggcatctcaggccagcaggcggggcccagagacccagaagcaccacaactcccccgtgtccacaaggcactttatgcattcaaaaccaccgaattcacacccaggtttgctcagacagaggcccagaggcgaccccgctctggcgtggctaccacctgagcggctggcggccctggcccagctcggcctccgcgtaggcgtcatacagcaccttcaggtgcaacagcagctgctccaggttctcgccggtcaacgccgacagcacgatgacctcctgtcccaagtgatcccggagctgggacagattggcttgggcttcagggaggtcaatcttgtttgcgacgattgcgtggggcctcgcagacaggcccttttcatacatctccagttcatattttaaatcgtcaacttgagtccacggctcaggctgagaaagatccaccacgaacaagagaaagcggcagcgctcgatgtgcctgaggaaggcggaccccagacccctgttctggtgggcgcctcgtatgatgccggggatgtcggccactttgggagaattctggaagttctacctgctatttgtaggtggccttcgtagtggacgatcccgacgtggggcttcagggtggtgaacgggtaggaagccacggcgggtctggcgtttgaaatggcccggagcagtgaggacttcccggcgttggggaatcccaccattccggcgtgggccaccgtcttgagctccaggtggagaactcgctgctgtcctggctgtccaggggtacaggtcacaggggcacggttgttgttggccaggaagaagcggttgcctttccctcctgccccgcccagcgcggcaatgtactcatctcccacgcaagacaggtcggccacaactctgcctccctccttcaccagcgtgcccacggggacccggatgtagaggacggcgccactgcgcccgaagcagtttttactccctccatcttctccactgaaaccctggtaccgcgacaggaccgacgacagggacttgacttgctggtcaactctcagaatgacgtgtccaccgttgcctccgtcccctccatcagggcctccaaactccttgcggggctcactgtggaagcagcttgccccagcgcctccgtttcctccacagacaagcactctccgatagtccacaaagtaccttttcagctttttctcagagagcagcttcttccccgggagttcctgatgcttggcgaggtccgcacggccgaccgagagcagcctgggagaagcccgctgtggcagtagccggctgggcttcaggccagcccatgtggacaaagcccaatgccccacgccctgaaacacggtcctcaatcttgctgagaaacaccttgcaggtgccatggccccggctcgggaaagcacgtcactt

SEQ ID NO: 10948 - RNA, 5009 nt, Homo sapiens
  source 1..5009: mol_type = other RNA
ctgaatagctgggactacaggtgaccgccaccacgcctggctaatttttttgtatttttagtagagacggggtttcactgtgttagccaggatggtctcaatctcctgaccttgtgatccaccagcctcggcctcccaaagtgctgggactacaggcatgagccaccgtgcccagaatgttctgtttttgtttgtttgtttgtttgttttttgagacagggtctcgctctgtcactcaggctggagtgcagtggtgcaatcacggctcactgcagccttgacctcccaggctcacatgatcctcccacgacagcctctggagtgtcccctccactttctttcttaggggcccctcagggacatgtcagaggcctgagactacttgggggatgtctatgggccaggcaggctgccagcagctgagctgtccttgccctggggctcctctgcagtcagggagacaccaggcatgggcctggcttggatgcatcagtacttgactgcaaagacttaaaccacagacaggaaaggcgctgctgcagtctcgacggtcaaatgcagggccccctcagctgccatcccactgaggggcgaaggcccatcatctcccttcggctcggtaactgcctggcgtagcacaagggttctctttaaatccccagcaaatggagctgagtggaaattccgccccatattaccaggcacacgtctccttccactcctcactataccctgcccatgccacggccgccttctgagaataacgctgacagttccatggcccacagcccctctagttaacttgctgtgcacacggcagcccagccagaaacacgcagccaggtcggatattgggtgcattcagtcgtgaagcctgaggcttcctggctcccactgagcacagagaagtgttctgaaggacaggaagcagctggcctcactgctcttctcagacggctgatggagaaaagctcacagctgcctgcgccgctctgcctggacttgcatcctcggccccaccccttgcgcagcagtgaggccccccgagacactggtgcctgggcttgcggtaccgcagggctgctggacaacgggccagacgcagccccagtgtggatccagaggtctctctccgtagcaagccatggaagcacgacgggcactgtgctgagaaccctggtctgcacttctgacctggggctctggctgtgcggttctgctgagctcatccgagagtccacgcgtgcatggcggagacctgagtcagcggcagggccaccccgttatgggcaccccaaccccttattaggggtgttaatcagcacaaatgagcaactggctcatcagtcggtgcaggctgacaggtgcaggaaatacggagggcaggcggggtagggggcacggaatgcttcccaacatgagggcatctcaggccagcaggcggggcccagagacccagaagcaccacaactcccccgtgtccacaaggcactttatgcattcaaaaccaccgaattcacacccaggtttgctcagacagaggcccagaggcgaccccgctctggcgtggctaccacctgagcggctggcggccctggcccagctcggcctccgcgtaggcgtcatacagcaccttcaggtgcaacagcagctgctccaggttctcgccggtcaacgccgacagcacgatgacctcctgtcccaagtgatcccggagctgggacagattggcttgggcttcagggaggtcaatcttgtttgcgacgattgcgtggggcctcgcagacaggcccttttcatacatctccagttcatattttaaatcgtcaacttgagtccacggctcaggctgagaaagatccaccacgaacaagagaaagcggcagcgctcgatgtgcctgaggaaggcggaccccagacccctgttctggtgggcgcctcgtatgatgccggggatgtcggccactttgggagaattctggaagttctacctgctatttgtaggtggccttcgtagtggacgatcccgacgtggggcttcagggtggtgaacgggtaggaagccacggcgggtctggcgtttgaaatggcccggagcagtgaggacttcccggcgttggggaatcccaccattccggcgtgggccaccgtcttgagctccaggtggagaactcgctgctgtcctggctgtccaggggtacaggtcacaggggcacggttgttgttggccaggaagaagcggttgcctttccctcctgccccgcccagcgcggcaatgtactcatctcccacgcaagacaggtcggccacaactctgcctccctccttcaccagcgtgcccacggggacccggatgtagaggacggcgccactgcgcccgaagcagtttttactccctccatcttctccactgaaaccctggtaccgcgacaggaccgacgacagggacttgacttgctggtcaactctcagaatgacgtgtccaccgttgcctccgtcccctccatcagggcctccaaactccttgcggggctcactgtggaagcagcttgccccagcgcctccgtttcctccacagacaagcactctccgatagtccacaaagtaccttttcagctttttctcagagagcagcttcttccccgggagttcctgatgcttggcgaggtccgcacggccgaccgagagcagcctgggagaagcccgctgtggcagtagccggctgggcttcaggccagcccatgtggacaaagcccaatgccccacgccctgaaacacggtcctcaatcttgctgagaaacaccttgcaggtgccatggcccctacagaagtcaaattggcaaaatgagatacttggtttaatgctgggcatgaaacagaaactgaagacgagggcctcatgcagcaggtctttgtgcacgtttctgaaacaaacaagtgaactgatgaatccgattttcctggtcactcaccctctcggccctgggtcacgtcttgccctctgacccgtcagcctatctgtgacttgggagcaggatttctgtacaaaggatttaaaacatgaaatcttccacaacactggacacatcctcttatggaatagcaaggttccgctcaacgaaaatattaaaaaggaaatctgaagtgcaagtcaaaatttcttgaaaagaaaaacacccatttattaaaatgttatcaagagtgttatcctgtgtaattttaaagttgttacattggaacacaagaatattaaacatggggcatagcggctaagcacccaggctctggaaagtaactctaagggaaggccatccacctgtgtggcctcggcctcctcacacggctgggtgaggacgggctgagctgatccacacggctgcacaaccgcggccctggctgtggcaccgatagaatgagaagaacacacttggcccctgctcctggctcctgacacagagctctcagaacgctggtaatttcctgagtgacaggggcgataggggtgcctgacacagagctcctaaatcccttggacttcccaggtgacaggagagtcttctgttctaatgaggcacctcttggtgggctcctggatggccttgggagggggctggtcatcataaagaccaagccacgatgagaagcctggacctttcggccccacccccaccctccaaaaagggcagaggggctggaggctgagttcataactgatcatgtctccatgatgaggcctccatggaaatcctggaactaggggctctggaaagctttcagtttggtgaactcatccccgtgctgtaaggccagccacacaactccctggggacaaaggctcctatgcttaggaccctctgggcctcgcccgtgcccctcctcacccagctgcctgcctgtgcccgctgtggcatcctttatagtaaactggcaatgcaaaccaagtgccttcctgagttctgtgagccactaccgcaaatcatcaaacctgaaggggtcgtaggaactcccaatgtgtagccaagatggacagaagtgtgggtaccccagggacccactacttgcaattagcatctgaagtggggggtgactgagcccctaacgctggggtccctgataaccgcggcagggtcagactgaactgaattacaggatgcctggctggtgtctgcagaggactggcgaattgttggtgtggaaaacccacacatttggtgcctgatgtgtagtgtgggtggaaatatccccggagcgacagggttggcacagctgcagactctaagtgccagctactgtcactctcaaagcctcatttaagctgtcactcattcaacaagccgctcatgacagccggctaccttgcaggtgccaagggcacagtgaggaagtcctgaccctgccctccaggagaggacagcccctctcccttcaccatgagcacaaatacctgcctgctcccagagctccccagtcttcagcaggtcgcacaggagggaccttacaaggtgctccccatcctgactacaaaagatgtgtacagaaggggccccagtggacggctgaaaactcaacacggggccagagcgggagcacaacgaggggacaccgcctgcctcctccctcgcagtgcctcggacgcctccctctccccagcctcactcctctgaaaaggtgccacctcctttgggggggtcactatctctgtggggtccttggccattctgctttaattctgaggcaatcacagttacagaaaagctggaagaagagtacaaagaacttcctcctgaatcacttaagagtcagtcgccgactggacttccctgcacccagaacagtccatgtgtgtttcctagagaaaatggtgtcccctccagaaccagggtgtcattgagactggccatgaccgacagcccctcccacgtgggccccggtctcagcagtgcctctccctgtaggaaagtctgcgtccctatcccggctgcctgcagctgccacaccttgtccagctc

SEQ ID NO: 10949 - RNA, 2277 nt, Homo sapiens
  source 1..2277: mol_type = other RNA
ctgaatagctgggactacaggtgactgccaccacacccagctaattttttttttgtatttttagtagagacggggtttcactatgttggccaggctggtctcaaactactgacttcgtgatctgcccacctcggcctcccaaagggctgggattacaggcgtgagcctccgcgcccgaccctttttatcattctatcaacataaccagtgttctcctttcatcttagactcaaacgcttaatgtattagtcaaccagttgcttgtctaactttattctttaatttgttaacaaaatctaccagttactctttttctacatgttttagatataaccattatttccatttccactcactttatttcagctcaggtcttaatttagtcttcttttttcacaaatgtttcactaaacatttgtgaaatgttaatctctgcacttataatttccctgtttttaacctatttacctccccagacaacgagtaacttaataaaattccccacttcctacttgtcaatctgcaaataatatcatgtcagtgaatgtgctggtgattcaggcaattatacagatctttataaaacttcatgtcttggcaaaaatgtattattgactggtggtaaaatatttgcataggaagttatatatagtgtaagtaatacatatgtgtgtgtgactgtgactgtgtgggtatgggtggatggtacaaatcatgcccaactgtaactattaagaatgctaaaaaaaaaaaaaaaccctaagaaccaaatattatcaaactgtcaaagtttaactcaactttcagccagccttctttttttctgtatttgcacagttataatcaaacagttaaatcttgcttactacatgttgactttccagcagagatgtgtgtggtcataatataaaacaagaaaaataggagtctatcatatctacaaatagaaggagaatattaaggtggacagaagcagcagaaacaaaatattcttatcaggcgaataaatctaatgtaaaaccagcaggctgtggagagaatagaaatttttccagtagccccttaacaagaccttggccttctggatccttggctgtgaatcagagtgttctggacacgtgattcttataaatcaatgggaggagacatttcccctgggtcttccaactcactgtaagtagctgaatatatgtttaattcttcataaacacgatcctctggaaccttgtttcctttgagttcttccccagctccacagattgtgagtgacacagcactaccaagtcccagaatggtgagaaacagcatcatcactacaatttcagtggaaaaggaagccataaagcacttggtctcaaaaaatttctggcaactgtggatgtggatataggccaagctcttcttcaggttgatgatcaggatggtaattcccgttcccccagctatgctgctggcagtgtttgctcccaggcttcctctcaccagatatgttgcatttctcctttcagatataattgacaacattccagaaatagaaaaaaatatggctccccagaatggataacctgctttaaatgatgaaaaaatgtctccctcaatgtgtgaaatatcaagtacagagcagacaactgttccaaaacaaaggcatatcatagcagtcagaatttgtgttacccccaggaactcctgctcttttttcaaaactgtcagccatgtatgcagtggtggggatgaggccgacttcaatagtctgcctgaagatacttcctggggagatatttccaagacttcaaatgcaggcacactggaaggctcctgtgggagagcaagatttgctctcctattactttctgtgtccattttttcattaaccgagctcatgacattgatgattctctttatacataagtcatttgccagacagataagtttcttggctgattaagatcaacaggcttttacttgtgatgaatagaaaaattaagaagtctactaaataaagactaatatgaaataagaaaatttgagactcctggagcataattttgcctgagactagcaggatttacagaacctgaaaatgagacattttagtaggagttgagaaggtgagaaagaactgcagaaaagaaagagatgtgcccttcttctggaattgtccccacttgtgtcccaattcagccatttctatggcagaagttatccaattgcacctttgaaaagcttgtcttccttgtttaaggcatgcttggtttcacacatagacccaaaactgaa

SEQ ID NO: 10950 - RNA, 1962 nt, Homo sapiens
  source 1..1962: mol_type = other RNA
ctgaatagctgggactacaggtgactgccaccacacccagctaattttttttttgtatttttagtagagacggggtttcactatgttggccaggctggtctcaaactactgacttcgtgatctgcccacctcggcctcccaaagggctgggattacaggcgtgagcctccgcgcccgaccctttttatcattctatcaacataaccagtgttctcctttcatcttagactcaaacgcttaatgtattagtcaaccagttgcttgtctaactttattctttaatttgttaacaaaatctaccagttactctttttctacatgttttagatataaccattatttccatttccactcactttatttcagctcaggtcttaatttagtcttcttttttcacaaatgtttcactaaacatttgtgaaatgttaatctctgcacttataatttccctgtttttaacctatttacctccccagacaacgagtaacttaataaaattccccacttcctacttgtcaatctgcaaataatatcatgtcagtgaatgtgctggtgattcaggcaattatacagatctttataaaacttcatgtcttggcaaaaatgtattattgactggtggtaaaatatttgcataggaagttatatatagtgtaagtaatacatatgtgtgtgtgactgtgactgtgtgggtatgggtggatggtacaaatcatgcccaactgtaactattaagaatgctaaaaaaaaaaaaaaaccctaagaaccaaatattatcaaactgtcaaagtttaactcaactttcagccagccttctttttttctgtatttgcacagttataatcaaacagttaaatcttgcttactacatgttgactttccagcagagatgtgtgtggtcataatataaaacaagaaaaataggagtctatcatatctacaaatagaaggagaatattaaggtggacagaagcagcagaaacaaaatattcttatcaggcgaataaatctaatgtaaaaccagcaggctgtggagagaatagaaatttttccagtagccccttaacaagaccttggccttctggatccttggctgtgaatcagagtgttctggacacgtgattcttataaatcaatgggaggagacatttcccctgggtcttccaactcactgtaagtagctgaatatatgtttaattcttcataaacacgatcctctggaaccttgtttcctttgagttcttccccagctccacagattgtgagtgacacagcactaccaagtcccagaatggtgagaaacagcatcatcactacaatttcagtggaaaaggaagccataaagcacttggtctcaaaaaatttctggcaactgtggatgtggatataggccaagctcttcttcaggttgatgatcaggatggtaattcccgttcccccagctatgctgctggcagtgtttgctcccaggcttcctctcaccagatatgttgcatttctcctttcagatataattgacaacattccagaaatagaaaaaaatatggctccccagaatggataacctgctttaaatgatgaaaaaatgtctccctcaatgtgtgaaatatcaagtacagagcagacaactgttccaaaacaaaggcatatcatagcagtcagaatttgtgttacccccaggaactcctgctcttttttcaaaactgtcagccatgtatgcagtggtggggatgaggccgacttcaatagtctgcctgaagatacttcctggggagatatttccaagacttcaaatgcaggcacactggaaggctcctgtgggagagcaagatttgctctcctattactttctgtgtccattttttcattaaccgagctgtccaggaataaagaatattattatattgagacttggtggatttcctcttactgcatgctctgaataggcagttgaaatgggtt

SEQ ID NO: 10951 - RNA, 1895 nt, Homo sapiens
  source 1..1895: mol_type = other RNA
ctgaatagctgggactacaggtgactgccaccacacccagctaattttttttttgtatttttagtagagacggggtttcactatgttggccaggctggtctcaaactactgacttcgtgatctgcccacctcggcctcccaaagggctgggattacaggcgtgagcctccgcgcccgaccctttttatcattctatcaacataaccagtgttctcctttcatcttagactcaaacgcttaatgtattagtcaaccagttgcttgtctaactttattctttaatttgttaacaaaatctaccagttactctttttctacatgttttagatataaccattatttccatttccactcactttatttcagctcaggtcttaatttagtcttcttttttcacaaatgtttcactaaacatttgtgaaatgttaatctctgcacttataatttccctgtttttaacctatttacctccccagacaacgagtaacttaataaaattccccacttcctacttgtcaatctgcaaataatatcatgtcagtgaatgtgctggtgattcaggcaattatacagatctttataaaacttcatgtcttggcaaaaatgtattattgactggtggtaaaatatttgcataggaagttatatatagtgtaagtaatacatatgtgtgtgtgactgtgactgtgtgggtatgggtggatggtacaaatcatgcccaactgtaactattaagaatgctaaaaaaaaaaaaaaaccctaagaaccaaatattatcaaactgtcaaagtttaactcaactttcagccagccttctttttttctgtatttgcacagttataatcaaacagttaaatcttgcttactacatgttgactttccagcagagatgtgtgtggtcataatataaaacaagaaaaataggagtctatcatatctacaaatagaaggagaatattaaggtggacagaagcagcagaaacaaaatattcttatcaggcgaataaatctaatgtaaaaccagcaggctgtggagagaatagaaatttttccagtagccccttaacaagaccttggccttctggatccttggctgtgaatcagagtgttctggacacgtgattcttataaatcaatgggaggagacatttcccctgggtcttccaactcactgtaagtagctgaatatatgtttaattcttcataaacacgatcctctggaaccttgtttcctttgagttcttccccagctccacagattgtgagtgacacagcactaccaagtcccagaatggtgagaaacagcatcatcactacaatttcagtggaaaaggaagccataaagcacttggtctcaaaaaatttctggcaactgtggatgtggatataggccaagctcttcttcaggttgatgatcaggatggtaattcccgttcccccagctatgctgctggcagtgtttgctcccaggcttcctctcaccagatatgttgcatttctcctttcagatataattgacaacattccagaaatagaaaaaaatatggctccccagaatggataacctgctttaaatgatgaaaaaatgtctccctcaatgtgtgaaatatcaagtacagagcagacaactgttccaaaacaaaggcatatcatagcagtcagaatttgtgttacccccaggaactcctgctcttttttcaaaactgtcagccatgtatgcagtggtggggatgaggccgacttcaatagtctgcctgaagatacttcctggggagatatttccaagacttcaaatgcaggcacactggaaggctcctgtgggagagcaagatttgctctcctattactttctgtgtccattttttcattaaccgagctttgaaaagcttgtcttc

SEQ ID NO: 10952 - RNA, 1827 nt, Homo sapiens
  source 1..1827: mol_type = other RNA
ctgaatagctgggactacaggtgactgccaccacacccagctaattttttttttgtatttttagtagagacggggtttcactatgttggccaggctggtctcaaactactgacttcgtgatctgcccacctcggcctcccaaagggctgggattacaggcgtgagcctccgcgcccgaccctttttatcattctatcaacataaccagtgttctcctttcatcttagactcaaacgcttaatgtattagtcaaccagttgcttgtctaactttattctttaatttgttaacaaaatctaccagttactctttttctacatgttttagatataaccattatttccatttccactcactttatttcagctcaggtcttaatttagtcttcttttttcacaaatgtttcactaaacatttgtgaaatgttaatctctgcacttataatttccctgtttttaacctatttacctccccagacaacgagtaacttaataaaattccccacttcctacttgtcaatctgcaaataatatcatgtcagtgaatgtgctggtgattcaggcaattatacagatctttataaaacttcatgtcttggcaaaaatgtattattgactggtggtaaaatatttgcataggaagttatatatagtgtaagtaatacatatgtgtgtgtgactgtgactgtgtgggtatgggtggatggtacaaatcatgcccaactgtaactattaagaatgctaaaaaaaaaaaaaaaccctaagaaccaaatattatcaaactgtcaaagtttaactcaactttcagccagccttctttttttctgtatttgcacagttataatcaaacagttaaatcttgcttactacatgttgactttccagcagagatgtgtgtggtcataatataaaacaagaaaaataggagtctatcatatctacaaatagaaggagaatattaaggtggacagaagcagcagaaacaaaatattcttatcaggcgaataaatctaatgtaaaaccagcaggctgtggagagaatagaaatttttccagtagccccttaacaagaccttggccttctggatccttggctgtgaatcagagtgttctggacacgtgattcttataaatcaatgggaggagacatttcccctgggtcttccaactcactgtaagtagctgaatatatgtttaattcttcataaacacgatcctctggaaccttgtttcctttgagttcttccccagctccacagattgtgagtgacacagcactaccaagtcccagaatggtgagaaacagcatcatcactacaatttcagtggaaaaggaagccataaagcacttggtctcaaaaaatttctggcaactgtggatgtggatataggccaagctcttcttcaggttgatgatcaggatggtaattcccgttcccccagctatgctgctggcagtgtttgctcccaggcttcctctcaccagatatgttgcatttctcctttcagatataattgacaacattccagaaatagaaaaccccaggaactcctgctcttttttcaaaactgtcagccatgtatgcagtggtggggatgaggccgacttcaatagtctgcctgaagatacttcctggggagatatttccaagacttcaaatgcaggcacactggaaggctcctgtgggagagcaagatttgctctcctattactttctgtgtccattttttcattaaccgagctgtccaggaataaagaatattattatattgagacttggtggatttcctcttactgcatgctctgaataggcagttgaaatgggtt

SEQ ID NO: 10953 - RNA, 3174 nt, Homo sapiens
  source 1..3174: mol_type = other RNA
ctgaatagctgggactacaggtgagaaccaccgaacgtggctaatattttaattttttgtagggacagggtctcactttgttgcccaggctggcctccaaatcctggcttcaagagatctttctgcctcagcatccccaaaagtgttgggatcacaggtgtggagccaccgtgcccccacgccgtcatggacctttttaatgagtataacaggctgacaacatctgaatctttatcaatcttaacatcaaaaaagagagaaaaccagaatgtctcaagcttcctgacatgacacaacaggaagcacaaagcaccacccgtatttaaacagaacctgaatctaatccagcaagtaaacctaactataacttacaagtatgaatgacagtgaaatacagcaaatgataccatgagaaaggcaatcaaccaaatctagaatatgggatatgtaagacaaatgacctttcaacaaatgactgtttttttgaaagggaggggagagttattgttctagattaaaataatgagacataaccatcaacttatggagatataacaaccaattatttggtgtgaaccttaactggatctatactcaaataaaccaaacacaaagacttcttttggataatgggggaaatgtgaatgcggactgggtatcagatattatgttatgaggttttgtgtgacatggcactgcgatgacttcttctgtttacgtgttttaaatagagatgcacactaagatatttacagatgaaacagtaagtctggaatgtgccttaaaaaaactcatagagggtgtggcagctcacacctgtaatcccagcactttcggaggctgagacaggcagattgctagagctcaggagttcaagatcagcctggacaacatggcaaaatcccacctctagaaacctcccccaaacccccgcgtgtgcgcgcgtatgcacacacacacacacgcacacaaaatcagctaggcatggtggcacacgcctgtagtccttgccactcagcaggctgaggtgggaggatcacttgagcccagaagttcagcttgcgcaacacagtgagatcccctctcttaaaaaacatcagaaaaatactcagagtaatgacatgtaagagacacataaggaacccggaagttactttgtgcatgactgaaaacattctagtgttttctaaagtaacttgccttgatttatatatgctcctacaaatatagaaacaaaggaccaaactaaagaggattaaaagtaataagagggtagaaaaagcagagaatttagggattcaggaaaaacaggttccaatataaactaactacatggtcttaggcaagccattcaacctctcaagtatgtttcctcatgttaaaacaaggttaagcccaggtgtggtggctcacgcctgtaatcccagcactttgggaggctgaggcgggtggatcacgaggtcaggtattcgagaccagcctggccaacatggtgaaaccccatctctactaaaaatacaacacttaggcaggagtggtggcaggcgcctgtaatcccagctactcagaaggctaaggcaggagcatcagttgaacccaggaggcggaggttgcagtgagccaagactgtgccattgtactccagcctgggtgacaggatgagactccgtctcaaaaaacaaacaaacaaacaaaaaaaccgcacaaggttaactcccatctcataggattatggaaaatttaaattaagtaagattgaaagtgctctcatttcattcaccaatttgaaagccatttattaagtagccattaggtagcacacacataatatacataaaagagcattactgtgattaaaaatgaaatgagtaatcaaattccaattcaatctaatttaaacttaccatatgggctaaaaaagtcacacgttttaagagaggcttcataattagtaacaagttcctggattatagaaacctgggacaagagtcaaaggtaatcttctgggtgtaattgctttggggtgctgcttactaatttcttcataaatttgaagcctctcttctaaagtgctaatttgtagagctttttccaagccttcataataacaccaattttctgcatttcgatcaatcaagtttttgaacacttcactggcttcttttaatcttcccaatttcaacagtatttcccctttaatttcttccaccaaaagtttatcacatatttgtttctcatacatttctatatgttccaaagattcctgcaacagatctgcctctctcatcacttgattctggtataatatcaattcactatattcataatctattttgtttggaggaacttgctgagtttgtctaaattcttccaacagttttagggccatatcataatctttcagcaaatggtatgcaatagcatatccaatccaggaggcacgctgtgtggggcgcaactgaagaagctggtatcttgtctctcggtaaccttcaaggtctctcatttggatctgcaacagtgagagatccctcaaaatttgcaggttatctttatctaatttgagggcatttcggtaacattttatagcttcatcatattttttatcagaacgctgcaagagtccatatacatgccaacagacatgactcttgacatcattacgaagtcctttacgaacaaactcataagcttcttctttttttcctaaacagttcagtgttaatcctttcatagccaaagtctctccatgttcagcaaattttgggttcgacagaatcatcttgcaaaacttgaggccatttttgtactgcttctgttcataacatttcaagatgcgtttgaagaggttgctctccttgggcggcagcagcacgttcggcatcgtggccggcagggaggctaggtggccggcagggaggctaggtgcccgggcgctccgcttcgcgggggtgggcaccgggacgaaccgctgctgagagtcgggctgcgggcgatggattagttcattggtctacagttgcaattgggcagcctggctgttcggcacgggtggcaatggagaaggaaggcggtctgagcaggacacgcttcccctgggctccgctttttggccagcggcggcggcggcggttcccgcgcactgcaagatggcagccagggtccgcctcccga

SEQ ID NO: 10954 - RNA, 5231 nt, Homo sapiens
  source 1..5231: mol_type = other RNA
ctgaatagctgggactacaggtgagcaccaccactccctgctaatttttgtatttttagtagagacggggtttcgccatgttggccaggctggtcttgaactcctgacctcaggtcatccacctaccttggcctcccaaagtgctgggattacaggtgtgagccactgcacctagcccagaatgttttatttttcttattatgggttgtatttttctgttgcatgcctggtaatttttgattggatgccagccattgtgaattttactttgtagattattttcatatccctaaaacagtttgaactttcttctggagtatgattaagttatttggacacagtttgaatgtttttgggtctctcttttaagctttgttaggttattctagagcatttagtcgagggttaatttttcccgctattgaagcaagacctttcttagtactctaactggtgccttgtgaattaggatcttttccactcttgctgacgggatcaggaatcattcaccatcctgtgtgagctttgagtattgttttctttaatcctttctgatggttctttgccaagcctttggttatttcctctcatgcatgtactaatcattatttagcttaatacttcaggagaatggtcagcagatctctggagttctctctgtgtcactctgtcctctctagtattctaccctgtgaactctagttgccttgggctctcaggactcccacttatatctcctcacctcacagagtcttctgggttccctctccccatgccaaagcctttcttcaggcagcaagttggagcaattgtattgctcaccttgtttgcattccatctctcatggattactatccttcactgcctatgtccaatgccttcagggccattgtttcatatattttgcccatttaaaaaaagtatttggaagtttataattactttctacttaaatttactagctgtcacaatcattactgaagaaattcactcttgcaataatatacatatgtacttcatttgacacagaatttcaacatgtaaagcatataagaatttcttgccacaatcatgtttagaatgcttacctataaggtgaatattaaaatattagtaaatacaatgacttttttcagattagacatgataaataacctgcaaggttacttgaccattggtcacacagaatttcagagagatcagaaccagtgtcaaaataggtatttgtctttttggctttttaaaggtcaaggttgaatcaagggtaaacgaaaatattgcatgaacatgaagctaaaattgaattttatgtaacacaacaacagcactgggtaaatagagataggtggatagactgtctcagtttctttttaataatttttatttttttaatcgaagctttacacataatttaaaaactcaaaggtaacaaaacctaatatgaaaaaagcccaccatgatgaagcagctgttctgcaggtgttttgccctcattctgtgtgtctactttcaattccaaatgggcttatatgaccaaagagatgcaggatctaaccaacatgtaccaacaggaaccatgagcatgtgtatggaactgggtcctgagagtgctggacaagaattaagtttgtgtttatataggacagcagtacccatttatagtattggcttagggttatgttaactcttccacactgcgtcataatccgaagagatctagaccatctaaacatcccacataatgtcacaatgacctaccacattgatgacatcatgctagctggataaggtgaataataagcagctagcatactgtacactggaggatgggaaataatccttaagacccagcaagctgttacctcagtgaaacttttagggcccagtaggctgcttgaatgccaagatatccccttcacagtaaaggacaaattattgcatctcacccactcatttcaccaaaattattctgccaccagggaagcacaccaagctgtgtaggcttctgtgggaattcagaagttggcagtactgttctgactcgtaaactgggtgagatagaaatctgccagttttcagtgggatccatagcatgtaaaagttctctagcaggtatggtgtatttagccctgttgcatggaccaattcaggatattctatgggacaagagtaaatgtgataagaagccatgaaagttgaaggcaagctccaatgggagaatcacaaggtcgactcctggcattctgtggcaaggctgggccatctgcagtgcaaaatcccaaaaacaactctatccatgctaatgtgccttggtaagaactgattatggacatcaagtgaccatgtagccagagaggcccatcatgagctgggcaaaggcaggtggtcaggctcccatgtcatatctgattctttaccaatgtcccttcctcagctcacaattatggccacttgggaggctctcatgtctagcttatggaggacaaaaaagcctgagctgaattcactgaggtttcttggaatataggttcaaaacaaaaatggactgctactgccctacagccccacacaggactggccttaaaagacagcagtaaggagaaccctcccaaaaggcataatgtggggcagtattcctggtcatcaactgtgtgtggaaagaaagtgtcttgaactaagaacatattttcatggcaaataagttggctagttgatcaggggtctggaataagactggtatatcagggacaagaagtctggagaagcagaggagaaatatatcagatatggcacataaggagggctttttgtattgtataacacaatctttatctgccagagacaatccaacatgtaagcagcattaaataaccaagtagacagatttagccagtaaacttcagcagctacaaccatcggctccaccgccccctccctccgcccccaggaatggcacagggggcttatgacaaagtagtcatcttgcaggaatgcaagtgagcaagaagccaatagatagcctccacttatccaatagccactccccaggctgggcgcggtggctcctgtctgtaatcccagcactttgggaggctgaggtgggcggatcacctgaggtctggagtttgagaccagcctgaccaacatggagaaaccccgtctctactaaaaatacaaaattagctggccgtggtggcgcatgcctgtaatcccagctactcacgaggctgaggcaggagaatcccttgaacccaggaggcagaggttgcagtgagccgagatggcgccacggcactccagcctgggcaaccagtgaaactccgtctcaaacaaaacaaaacaacaacaacaacaacaacaaaatagccactccccagtgttaaacaccaagttcctgatacagcaccaaccctcaaggataccaaacagctacttgggcagcaaattgatttatgttggattccttccatcctagaatgggcagtgattctccttgactagaaactgcccatctgcatgtatgagtttgacttccttgcctataagttgttggccagctctactactcacaggtttacaggtatttgatccatcaacatgtatcctgtgtaatattgcctttgatttagggatgcactttacagcaaaggaggtgtatcagcaggtacataaccatgagatccactagtcctatcacatactatataaccgagaaaatgcgggtctgatggaatgatgaaaaacccttttgaaggtgaaactgaagcaaaagcttgaagataatagcctgtgaaaatggaatgaccttgtccaccagggtacagtatatactctaaatcaacactcattttatggtgctgtgtctcatatatacataacatgcatgtttgggaatgaaaggatataaatagaattcctactgtgtagtaggctgaataatggcccccaaatatgttcagatcctaatcctggattctatgaatattttaccttcaagataaaagagactttgtggatatgactaagttaatgatctcaagatacagagattatcctggactatccaataggcccaatataatcataaagattcttacaagagagaggcagatttgcctagtagatgcaatgacttaagcaggaggatggggtgatatgagtaaggggccatgagccaagaaatgtaggtagcctctagaaattgaaaaaggcaaggaaacagactttttcttgaagacttcaggaaaaacagtccagttgatatcttgattttaggcttccagaactgtaagaaaataaatttgtgttgtttgaaaccactaagttcgtagtgtcatagcagtgataggaaattaatataaccacatactctcactcccagtgacccaagtggggagtttggacttctcatccccgcaactttgtgaattagaagtcctgattcccaagagaggaaccttttcatcaagagacacaataatagatcctttaaactttaacttgctgaggtttcccggttcaaggtccttgtgctaggagaccagcaggcaaggaagagtcaccatgttagttggggtaaatgaatccaatcatcaggaggaaatagcgttattgctacacgatgatggcaggaaggaatatacctgtagtttacactcaagaccatatagtggtctcttgatatgtcccaatatcaagtaaagtggacaacttccaaaacagcagggtaaacatctccaaatactggcttctctcaaagatgagaaatatcaaagacaggaaaccctaggttcttgcccttcagtcgctatctccttgccattagtaaaatgcggccgatgaatgtcctcacttctgtccatctgggcaggaggtgggaagggtgacgtgcaaatggatgggaggaacccttttttcggcagcacccaccacacccagcctagtgccacgcaccgcaagcgctccataaacgcacacagcgtcgcctctaccaggatcccgggcggccttcgcgggatttctcctggcgtcggctttcagactcccgagggtgggataaatcgagagggtggcatcctttggcttttcttctcccaggcagctctgaaccatgtttatgcaacgtttaatgggctctaataaaacggctaataattttgatccgcggaagcaccgactcgctcgctaagccgaatctgcgagggtgaagctgcaactccaacgccggaaag

SEQ ID NO: 10955 - RNA, 1982 nt, Homo sapiens
  source 1..1982: mol_type = other RNA
ctgaatagctgggactacaggtgagcaccaccatgcctgtcttttttagaaaaacaaatttaaggttgaagccagaaaagccagattttcagcctgccagctacgcgtttgcaattttggtctatacaatttgagtagagactggagcagcaatcctgtctgaactcctacagtgcttatagcctgtgtcgcatcattagctcttagctactctttgtcttgctattcattagtttgtaaatcatttttcctaattagatgggacatagaacaggtgagaaatcatgtcttaaactttgtgtaccttaaaggtgcacaataggttttcagtatatactaggataaagactaattgattggctgattactcagaactatcactttctcctttgattttggaggagcaggtctggggaattcattattttacctcaccatttcagttttcccctctttacaaagagctcgggattcatcaatctccattaaacttcaaaatgaaatagtccacataagtcagagatgcaaaacccactgtattaattaggacttttctaattgcaagtaataggaaacccaaattcaaactgccttgggtaagacataatttactgattcctatagctaaaacctgcagaggtcaggatgatgtcaggcatgactgaattcaggaactcaggcaatgtcattggaacttgatctgtctttccctccgtggcttggctctacttttcctcccattagcttcactctcagtagttccctttcacgtggggcttctggcagcttctctttccagcagatccacaaaattcccagtcttgtgagattttcttgggatatgtgacgatctctcaatcagcccattgactagggctgggcgtgttaatcaggacttttctagttgtgataggaaacttaaattcaaactgccttaggctgagtcacttgtctgtccctaagagccagtggtaaatcagctccatccagcatccaatgtctgcataaaggacccagtttatggcttctccctctagccactcccagaggcagtgactacgtagaggggcctagtagggagtatgtggcggaagggaggccttgaagctgtgttcttatagcgtcctatatgaaactgaaaagcatcaatagcaaataacagagaagatctaatggagattatagagaggtagaggggactaaaggcctcccaagtcaccccttggtgccacccctgtaacatatttaatttgtgggggaagcaaaggcccagtaggactgctggtggcccagccacagtccaaaacaggccctagagaggacgcgctctaaccacacaccctaattattagtccctgaatatagatcagtttagtttatccaaagccccagctgaagacacatcaagtactattgcctctgttccatgttttgttccatataaacatccagacacaggtctcatgggagaaacatcatgaggcagtttcacagtccctggctttgatctttacgctgtagtaaaggtgtcattggcctttctggggcgaagagtcatgctcttccacaagagtatcaaattactgctcattttccaatgtatattctttcagggccttgctttcttcttacctgcccacaccaatgctgtgagggagactgctgatggcgaaggtgaaaatggtcaggcaatgtcattgggacttggtctgtctctccttccattagcccacttcttttatccagaaagatttcactgcaccgctcagtcctgaagtgtccaaggatgaaactgtgcggaaattctccctgtcgctctcagtttgtgggggaagcgccgggactgaggtacatggttaacacaggctgtgcgtgaaggggcttttgacttttcccccggctccggcctctcgcgtctctctcctagggctgcggctgctgctgcctggcgggcacaagccgggcggcggtgcgcggggggt

SEQ ID NO: 10956 - RNA, 9060 nt, Homo sapiens
  source 1..9060: mol_type = other RNA
ctgaatagctgggactacaggtgagtgccaccacacccagctaatttttgtatttttagtagagatgggggttcaccatgttgcccaaaatggtctcaatctcttggcctcgtgatccaaccatctcagcctcccaaagtgctgggtttaaaggcatgagccactgtgcctggcccagaattctttactgctaacacgagtgggcctggttctggaggatttcccagtgggtcctgaagaaccacagtttattggcttgtgggcaaaggggtatgtgtatcagttggcctttactgtgtaataaacagccacaaaaattactagctgaaaacagcagctacttaattagcagaagcctcttgaggatggacttgcaaaccaaagttgtgctggtttctactggtcaaagcaaggactggctcacataaaaaggagagagattgcaccttcagagagtaatctcaagacatctgtaatctaccacagggtgtcactgggcctctgtcaaggagcctattctttctgccaccagatctgtctaatagcttgtgtgacaatgcacttccttctgggtctctctccaagtgtagtaagtgtatatgggaatcactttattcaaacagtgtagtgcacttagttagaaagaaaaggtattaaggaagacttatatttaaaattgttatttatggtaacaacgaaaagtaacatacaaatttcaaacatcaagaataaaataaattaaaggtatgatcaatacacatcagtacaaagaggggaacacaatgaaacaaacaaaaaaaattagatgctagaaattaatccaaattattactaattaaatgtcaggcactaaatgtgcaacataaaaggattgttaattggtattattcaagtattttttctttttttttttttttttgtgacagagtttcactcttgttgcccaggctgcagtgcaatggcgtgatctcggctcactgcaacctctgcctcccgggttcaaatgattctcctgcctcagcctcccaagtagctggcattacaggcatgcaccactaggcacagctaattttgtatttttagtagagatggggtttctcagtgttggtcaggctggtctcgaactcccgacctcaggtgatcacctgccttggcctcccaaagtgctgtgattacagacatcagccactatgcccagcggtatacagattttttaaaactccagctaaagtatgtataaaaagacacatttttttaaaaagcatacagaaagactaagaagtagaggaaaatcaagctgatgtaactatataaatatctaacagaattagtggaacagaaaacatgcaagaaatagtgtagatttttcaagcgaaatatctgaaagaattcataaacctgggtactctctaccaagattaacacaagcaaagggaaagaatgcacaattaataagttattccagaatgcaaaaggagactgaagttatacaaccagcaaaaatgaaaaatataaaaagtataaatttttgctacacatttggaaataaaaacatgcctagaagaatattctcaaaatacttatgcaagccttagttgtctttttttttttttttttatgagatggagttttgctcttgtcacccaggctggagtgcagtggcaagaactcaactcactgcaaccttcgcctcccagattcaagcaattctcctgcctcagcctcccaagcggctgggattacaggcgcccgccaactcacctggctaattttattttttgaatttttagtagagacaaaagtttcaccgcattggccaggctggtctcgaactcctgacctcaggtgaccccctgccttgacctcccaaagtgctgtgattaaagccgtgaagcaccgtgcccaacctagttgtctttttttttttttttgagacggattctcgctctgtcgtcaggctggagtgcagtggtgtgatctaggctcattgaaacctccacttcaggggttcaagagattctcctgcctcagcctcctgagtagctgggattacaggggcacaataccgtgcccagctaatttttgtatttttagtaaagacggggtttcaacatgttggccaggatggtcttgatctcttgacctcatgatctgcctgcctcagcctcccaaagtggtgggattacaggcatgagccaccactcccagcctgataactgttttatttatttatttttatttttttggagatatggggtctgtgttgcccagactgatcttgaactcctggcctcaaggaatccttctgactgagcttcccagtgtgctgggattaaaagtgtgagccactatgaccagccagaagagataattttaactttttaaaatattttgcagtattggccgggcacagtggcttgtgcctgtaatcccagtactttgggagtatgaggcatgcagatcacctgaggtcaggagtttgagaccagcctggccaacttgatgaaaccgtctctactaaaaatacaaaaatcagccaggcaaggtggaggctgtctgtaatctcagctactcgggaggctgaggcaggagaaccactggaacccaggaggtggaatttgcagtaagttgagatcacaccattgcactccagcctgggcaacgagtgaaacactaactcaaaaacaaagaaacaaacaccaactcaaaaacaaagaaacaaaccaaaaaaatgaaaatatcttgtagtatttttaaatagagatgtggtttcgctatgttgcccaggctggtttgaactccttggctcaagggatctttttgcctcagcctccaaaagtgctgggattacaggcctgagccactattcccaacctagatgactcttatagattaagaatttagaaatagtaggaacatgccccactacagtatatgacagtcattatatacaaatatcattaagggacaattttttaaaaatcacaatgttattcaaacatagctccataacatattagtaaaggtcatgaagtatttttaagtgatccattatgtcacagtcgagcttatccaggaatacaaggttgatgtaacattggaaaagcaataaatacaaataccacatttatttaatttaatttatttatttttgacagagtcgcaccctgtcacccagcatggagtgcagtggtgcaatcttggctcaatgcaacctccacctcccaggttcaagtgattctcctgcttcagcctcccaagtagctgggattacaggtgcacatcaccacacccagctaatttttgtattgttagtagagatggggtttcaccatgttggctgggctggtctcgaactcttgacctcaaatgatctgcccacccccacctcccaaattgctgggattacaggcataagcccccacacccagcctgaccacatttgttttagaaaagcgcctttccatgcattcacttcttcaagttttttttttgttttgtttttgtttttttttttgagatggggtcttgctatgttgcctaagctggtctagaacccctgggctcaggccaccctcccaagtagctaaaactataggcatgcatcaccacatcatttcattgaagtatttattaggtaccatcatgagctaggtgcagttctaggtattgagttttatcagtaaataaacatgatcatcacagaggatgtgaaggaagcatttaataaattcaagaggaattcagcctcataaactatgaaatattgggaaataattcatcatgtaaaaactggatataaagaaaaaacttttcctgcaggacattgttgcaggaagtcagggaccccaaacggggggactggctgaagccatggcagaaaaacatggattgtgaaggtttcatggacatttattagttccccaaattaatacttttataatttcttatgcctgtctttactgcaatctctaaacataaattgtaaagatttcatggacacttatcacttccccagtcaatacccttgtgatttcctatgcctgtctttactttaatctctcaatcctgtcagctgaggaggatgtatattacctcaggaccctgtaataattgcattaactgcacaaattatacagcatgtgtgtttgagcaatatgaaatctgggcaccttgaaaaaagaacaggataacagcaatgtttaggaaacaagagagataaccttaaattctgaccgccggtgagccaggtggaacaaagccacatttctcttctttcacaagcaaatgggagaaatatcactgaattctttttctcagcaaggaacatccttgagaaagagaatgcacacctgggagtgggtctctgaactggcccccctgggtgtagccatctcttatggtcgagactgcaggggtgaaatagaccccagtctcccatagcactcccaggcttattaggaagaggaaattcccacctaataaattttagtcagaccagttgatctcaaaaccgtctcctgataagatgttatcaatgacaatggtgcccaaaacttcattagcaattttaatttcaccttggtcctgtgatctcgccctgcctccacttgccttgtgatattctattaccttgtaaagtacttgatgtctgtgacccacacctatttgcacactccctccccttttgaaaatccctaataaaaacttgctggtttttgcggcttgtggggcatcacggaacctaccgacatgtgatgtctgccccggacacccagctttaaaatttctctcttttgtactctgtccctttatttctcaagttggctgacacttagggaaaatagaaaagaacctatgtgaatatcggggctggttccctgacaggacataacctcttcaaaaaataaaaaagaaataaaagcctacagccaaaccaacaaaatagagtgcatatctcaccagaactgcaaagacaagtatgctggtattactacttttagttggtgttgtgcagcgggttaaaatcagtccagtaaagcaagaaaatatttagagagagcttcatcatcatacgaattttgggggtcattgttcagtccaaagtacttaatatgattcttttctctttccacatagagaatcagataatctataaataatgactcttactgttccactttaggagttaggtatacatacatatgtgtatatatatgtatatatatatacacatacacacacacacacacacacacacagtgaccccccaaatttcatatgaagttccaaacctcaatgtgactgtatgtgaaaagagaagggggcggggaggggggagaccgaccgacctatttgttggtctccatcgtgtgaaaacatgaggaagtgggcacttacatgccaggaagagagctctcactagaggttgaccatgctggcactctgatctcagacttccagcctccagatatgtgagaatataaatttgtgttttgggccagatacggtggctcaggcctgtaatcccagcactttgggaggccaaggcaggtggatcaccaaaggtcagatctgaccaacatggagatcagcctaaccaacatggagaaaccctgtctctactaaaaatacaaacttagctaaggtttgtggtgcatgccaataatcccagctactgagggtgaggcaggagaatcactggaactcaggaggtggaggttgcggtgagccaagatcataccattgcactccagcctgggcaacaagagcaaaactccatctcaaaaaaaaaaaaaaaaaaaaaaaaaaaatcctgtgtttttaacctcattgatttaaaattaaattaatttctaagccatttggtctgcggtattctcttatggttgtctgagctgactaaggcagatattggtactgagaagtgaggtactgcaattaaaaacaaacaaaaaaactaaaaatgtgaagcagctttgaaactgacaaatgagtagaggctggaaaaattctgatgtgcaagctggaaataaggttggtaagggttattctggtgaggtgtcattggggaatgaggaacatgctattgggaaatgaagaaaagacaacccttgatataaagtggtgaagaacttggcagaactgtattctagcattttacggaaggtagagcttgagacagataaaatggtatgtatcactaagatctgtaattaaagtgttaaaggacacaggaagcttcattattcctgagtgcttacaggaaaatgtgctgggaacaggccccccaaatctggccataaacaggcaatgagaaactggccataaacaaaatctctgcagcactgtgacatgctcgtgatggctatgacgcccatgctggaggctgctggtttaccagaatgagggcaagcaacacctggcccacccagggcagaaaactggaaaactgctcaaggcattcctaaaccacaaacaatagcatgagtgatttgtgccttaaggacatattcctgttgcagataacaagccagagcctgtccctttctttctcataaggaatacttatagctgatctacaatctataggaataatgtttatcacaggcttactgtcaataaatatgtgggtcaaactctgttcaagctcagctctgaaggctgtgagccccgattcccactctgcactatatttctgtgtctttgtcttaattcctctagagccactgggttagggtctccacgacccagctggtctcggcaaaaatgcaaaaggagacctgaattgcagaagaaattgttaaggaaaaaggaaccagaacttggagatttggaaaattctcagcctatccatactgcaaaaattagaaaacttgtactgaagagaatcctcaaagtgtggctgaacaatcatttgataaagagatcatgagtgggattcatggactatatcagccatcttaacagaagtgagaagagagactggattatactataagagacactgccacttacattgtgccacctaaaatggacagagaagacagaacagaacagtcaaggttgtcacacttcttattttacaagaaggggacatagaaataatcagctgtgaaagggcactggcagttatggatggtttcactcctgacatgctctgcaggatccatgggaacagaagagaaccttggaggagcatctttttaacaatccacctctggggcctacatcatcttggcttctggtaaattttgacatgaatgtgccacactggcagccactaaccaacaggggctgggatcaatctgcatgatttatctcgtacagaacttgttaatgctatgatcttaggaatctaatcaccaaggtgaggcagcctgcagtactgacctcaccatccatgacccttcttcacagatgcccagactcaggtaaccatgatgttgtattcagaacctgtaggtttaatttcagaccctcgggatgcatctaaggccaatctgtgagccattacaacctccaaaaggcatttaggactaatctgatgatctttgcactgccaataattaaagatggcaaccaatgggctaaatggtaacaacactcatatccttacattcatagtatttctccccagtgtgaattctttcatgcatacttaggcatgaggaaagagcaaatgctttcccaaattctttacatacaaaaggtttctctctggtaggagttcacaggtggggtgaggaatacagaaattctttcccacatatcttgcatttacctttctccactgtgagttttcaaatgtttactacgatgggaagaagtaatgaaggtcttcccacattcaacacattcataaggcttctctcctgtgtgaattcttctatgttgagtaagcgttgaagatctattgaaggctttcccacattccttacactgatagggtttctctccagtgtgatttcgtatgtgtatagcaaggcccgtgtactgagtgaaggcttggccacattccttacattcatagggttttattccagtgtgagttcttacatgttgagtaaggtgagttgatctagtgaaggctttcccacattccgtacatttgtgtggttttattccagtgtgaatttgaatgtgaacattaaaggatgaggaatttctaaaggatcttccacattctttacattcaaaggacttctctcctttatgagtttttgcatgtgcagaaagttgagaaaaattagtgaaggatttcccacagttcttagtcttttcggatttctttccagtatgaactgctacacactgctttaagtgtgaggaagttgtgatggctctctcacattcctgaaattcacagagtttctctccaatgtggattcccatgtgattatcaaggcttgcaaaatacttaaagccttttccacattccttacatttgtagggttgtcttccattgagaatttcaagatgcacagcaaggcctggagttaaggtgaagacttttccacatggattaaatttggaaagttcttgtccaatagaggcttccttgtgcacactgatgctgtcttttccataacaattaccctcaaaagtgttccctccattctgagctctcatgtgtgtcttaaggcaaaactgttcactgaagacctctccacaattctcacagagtttccatccactgtagcttcttgtctgcatttgtatcccagtgaatatttgattcttcaaaaaaccctgctgaagtgatgaccgtttggttctaggttgtatttcccattctgaagttaagcagaaaaagaaatcatgggacatatcaaaggctgacatcctctgaagctgatggtgagatgtgcctcaatgctgtctttcttgatgccaagatcgcctcagggcagcttatgaatctaggtggatacaggcaatctccattcccctttgtacagggttatctgaggcccacagcggggtggactccaccacaataaaggttaaacggcactgaccatgctgagccacagccggtaaagatggcggtggcacact

SEQ ID NO: 10957 - RNA, 9223 nt, Homo sapiens
  source 1..9223: mol_type = other RNA
ctgaatagctgggactacaggtgagtgccaccacacccagctaatttttgtatttttagtagagatgggggttcaccatgttgcccaaaatggtctcaatctcttggcctcgtgatccaaccatctcagcctcccaaagtgctgggtttaaaggcatgagccactgtgcctggcccagaattctttactgctaacacgagtgggcctggttctggaggatttcccagtgggtcctgaagaaccacagtttattggcttgtgggcaaaggggtatgtgtatcagttggcctttactgtgtaataaacagccacaaaaattactagctgaaaacagcagctacttaattagcagaagcctcttgaggatggacttgcaaaccaaagttgtgctggtttctactggtcaaagcaaggactggctcacataaaaaggagagagattgcaccttcagagagtaatctcaagacatctgtaatctaccacagggtgtcactgggcctctgtcaaggagcctattctttctgccaccagatctgtctaatagcttgtgtgacaatgcacttccttctgggtctctctccaagtgtagtaagtgtatatgggaatcactttattcaaacagtgtagtgcacttagttagaaagaaaaggtattaaggaagacttatatttaaaattgttatttatggtaacaacgaaaagtaacatacaaatttcaaacatcaagaataaaataaattaaaggtatgatcaatacacatcagtacaaagaggggaacacaatgaaacaaacaaaaaaaattagatgctagaaattaatccaaattattactaattaaatgtcaggcactaaatgtgcaacataaaaggattgttaattggtattattcaagtattttttctttttttttttttttttgtgacagagtttcactcttgttgcccaggctgcagtgcaatggcgtgatctcggctcactgcaacctctgcctcccgggttcaaatgattctcctgcctcagcctcccaagtagctggcattacaggcatgcaccactaggcacagctaattttgtatttttagtagagatggggtttctcagtgttggtcaggctggtctcgaactcccgacctcaggtgatcacctgccttggcctcccaaagtgctgtgattacagacatcagccactatgcccagcggtatacagattttttaaaactccagctaaagtatgtataaaaagacacatttttttaaaaagcatacagaaagactaagaagtagaggaaaatcaagctgatgtaactatataaatatctaacagaattagtggaacagaaaacatgcaagaaatagtgtagatttttcaagcgaaatatctgaaagaattcataaacctgggtactctctaccaagattaacacaagcaaagggaaagaatgcacaattaataagttattccagaatgcaaaaggagactgaagttatacaaccagcaaaaatgaaaaatataaaaagtataaatttttgctacacatttggaaataaaaacatgcctagaagaatattctcaaaatacttatgcaagccttagttgtctttttttttttttttttatgagatggagttttgctcttgtcacccaggctggagtgcagtggcaagaactcaactcactgcaaccttcgcctcccagattcaagcaattctcctgcctcagcctcccaagcggctgggattacaggcgcccgccaactcacctggctaattttattttttgaatttttagtagagacaaaagtttcaccgcattggccaggctggtctcgaactcctgacctcaggtgaccccctgccttgacctcccaaagtgctgtgattaaagccgtgaagcaccgtgcccaacctagttgtctttttttttttttttgagacggattctcgctctgtcgtcaggctggagtgcagtggtgtgatctaggctcattgaaacctccacttcaggggttcaagagattctcctgcctcagcctcctgagtagctgggattacaggggcacaataccgtgcccagctaatttttgtatttttagtaaagacggggtttcaacatgttggccaggatggtcttgatctcttgacctcatgatctgcctgcctcagcctcccaaagtggtgggattacaggcatgagccaccactcccagcctgataactgttttatttatttatttttatttttttggagatatggggtctgtgttgcccagactgatcttgaactcctggcctcaaggaatccttctgactgagcttcccagtgtgctgggattaaaagtgtgagccactatgaccagccagaagagataattttaactttttaaaatattttgcagtattggccgggcacagtggcttgtgcctgtaatcccagtactttgggagtatgaggcatgcagatcacctgaggtcaggagtttgagaccagcctggccaacttgatgaaaccgtctctactaaaaatacaaaaatcagccaggcaaggtggaggctgtctgtaatctcagctactcgggaggctgaggcaggagaaccactggaacccaggaggtggaatttgcagtaagttgagatcacaccattgcactccagcctgggcaacgagtgaaacactaactcaaaaacaaagaaacaaacaccaactcaaaaacaaagaaacaaaccaaaaaaatgaaaatatcttgtagtatttttaaatagagatgtggtttcgctatgttgcccaggctggtttgaactccttggctcaagggatctttttgcctcagcctccaaaagtgctgggattacaggcctgagccactattcccaacctagatgactcttatagattaagaatttagaaatagtaggaacatgccccactacagtatatgacagtcattatatacaaatatcattaagggacaattttttaaaaatcacaatgttattcaaacatagctccataacatattagtaaaggtcatgaagtatttttaagtgatccattatgtcacagtcgagcttatccaggaatacaaggttgatgtaacattggaaaagcaataaatacaaataccacatttatttaatttaatttatttatttttgacagagtcgcaccctgtcacccagcatggagtgcagtggtgcaatcttggctcaatgcaacctccacctcccaggttcaagtgattctcctgcttcagcctcccaagtagctgggattacaggtgcacatcaccacacccagctaatttttgtattgttagtagagatggggtttcaccatgttggctgggctggtctcgaactcttgacctcaaatgatctgcccacccccacctcccaaattgctgggattacaggcataagcccccacacccagcctgaccacatttgttttagaaaagcgcctttccatgcattcacttcttcaagttttttttttgttttgtttttgtttttttttttgagatggggtcttgctatgttgcctaagctggtctagaacccctgggctcaggccaccctcccaagtagctaaaactataggcatgcatcaccacatcatttcattgaagtatttattaggtaccatcatgagctaggtgcagttctaggtattgagttttatcagtaaataaacatgatcatcacagaggatgtgaaggaagcatttaataaattcaagaggaattcagcctcataaactatgaaatattgggaaataattcatcatgtaaaaactggatataaagaaaaaacttttcctgcaggacattgttgcaggaagtcagggaccccaaacggggggactggctgaagccatggcagaaaaacatggattgtgaaggtttcatggacatttattagttccccaaattaatacttttataatttcttatgcctgtctttactgcaatctctaaacataaattgtaaagatttcatggacacttatcacttccccagtcaatacccttgtgatttcctatgcctgtctttactttaatctctcaatcctgtcagctgaggaggatgtatattacctcaggaccctgtaataattgcattaactgcacaaattatacagcatgtgtgtttgagcaatatgaaatctgggcaccttgaaaaaagaacaggataacagcaatgtttaggaaacaagagagataaccttaaattctgaccgccggtgagccaggtggaacaaagccacatttctcttctttcacaagcaaatgggagaaatatcactgaattctttttctcagcaaggaacatccttgagaaagagaatgcacacctgggagtgggtctctgaactggcccccctgggtgtagccatctcttatggtcgagactgcaggggtgaaatagaccccagtctcccatagcactcccaggcttattaggaagaggaaattcccacctaataaattttagtcagaccagttgatctcaaaaccgtctcctgataagatgttatcaatgacaatggtgcccaaaacttcattagcaattttaatttcaccttggtcctgtgatctcgccctgcctccacttgccttgtgatattctattaccttgtaaagtacttgatgtctgtgacccacacctatttgcacactccctccccttttgaaaatccctaataaaaacttgctggtttttgcggcttgtggggcatcacggaacctaccgacatgtgatgtctgccccggacacccagctttaaaatttctctcttttgtactctgtccctttatttctcaagttggctgacacttagggaaaatagaaaagaacctatgtgaatatcggggctggttccctgacaggacataacctcttcaaaaaataaaaaagaaataaaagcctacagccaaaccaacaaaatagagtgcatatctcaccagaactgcaaagacaagtatgctggtattactacttttagttggtgttgtgcagcgggttaaaatcagtccagtaaagcaagaaaatatttagagagagcttcatcatcatacgaattttgggggtcattgttcagtccaaagtacttaatatgattcttttctctttccacatagagaatcagataatctataaataatgactcttactgttccactttaggagttaggtatacatacatatgtgtatatatatgtatatatatatacacatacacacacacacacacacacacacagtgaccccccaaatttcatatgaagttccaaacctcaatgtgactgtatgtgaaaagagaagggggcggggaggggggagaccgaccgacctatttgttggtctccatcgtgtgaaaacatgaggaagtgggcacttacatgccaggaagagagctctcactagaggttgaccatgctggcactctgatctcagacttccagcctccagatatgtgagaatataaatttgtgttttgggccagatacggtggctcaggcctgtaatcccagcactttgggaggccaaggcaggtggatcaccaaaggtcagatctgaccaacatggagatcagcctaaccaacatggagaaaccctgtctctactaaaaatacaaacttagctaaggtttgtggtgcatgccaataatcccagctactgagggtgaggcaggagaatcactggaactcaggaggtggaggttgcggtgagccaagatcataccattgcactccagcctgggcaacaagagcaaaactccatctcaaaaaaaaaaaaaaaaaaaaaaaaaaaatcctgtgtttttaacctcattgatttaaaattaaattaatttctaagccatttggtctgcggtattctcttatggttgtctgagctgactaaggcagatattggtactgagaagtgaggtactgcaattaaaaacaaacaaaaaaactaaaaatgtgaagcagctttgaaactgacaaatgagtagaggctggaaaaattctgatgtgcaagctggaaataaggttggtaagggttattctggtgaggtgtcattggggaatgaggaacatgctattgggaaatgaagaaaagacaacccttgatataaagtggtgaagaacttggcagaactgtattctagcattttacggaaggtagagcttgagacagataaaatggtatgtatcactaagatctgtaattaaagtgttaaaggacacaggaagcttcattattcctgagtgcttacaggaaaatgtgctgggaacaggccccccaaatctggccataaacaggcaatgagaaactggccataaacaaaatctctgcagcactgtgacatgctcgtgatggctatgacgcccatgctggaggctgctggtttaccagaatgagggcaagcaacacctggcccacccagggcagaaaactggaaaactgctcaaggcattcctaaaccacaaacaatagcatgagtgatttgtgccttaaggacatattcctgttgcagataacaagccagagcctgtccctttctttctcataaggaatacttatagctgatctacaatctataggaataatgtttatcacaggcttactgtcaataaatatgtgggtcaaactctgttcaagctcagctctgaaggctgtgagccccgattcccactctgcactatatttctgtgtctttgtcttaattcctctagagccactgggttagggtctccacgacccagctggtctcggcaaaaatgcaaaaggagacctgaattgcagaagaaattgttaaggaaaaaggaaccagaacttggagatttggaaaattctcagcctatccatactgcaaaaattagaaaacttgtactgaagagaatcctcaaagtgtggctgaacaatcatttgataaagagatcatgagtgggattcatggactatatcagccatcttaacagaagtgagaagagagactggattatactataagagacactgccacttacattgtgccacctaaaatggacagagaagacagaacagaacagtcaaggttgtcacacttcttattttacaagaaggggacatagaaataatcagctgtgaaagggcactggcagttatggatggtttcactcctgacatgctctgcaggatccatgggaacagaagagaaccttggaggagcatctttttaacaatccacctctggggcctacatcatcttggcttctggtaaattttgacatgaatgtgccacactggcagccactaaccaacaggggctgggatcaatctgcatgatttatctcgtacagaacttgttaatgctatgatcttaggaatctaatcaccaaggtgaggcagcctgcagtactgacctcaccatccatgacccttcttcacagatgcccagactcaggtaaccatgatgttgtattcagaacctgtaggtttaatttcagaccctcgggatgcatctaaggccaatctgtgagccattacaacctccaaaaggcatttaggactaatctgatgatctttgcactgccaataattaaagatggcaaccaatgggctaaatggtaacaacactcatatccttacattcatagtatttctccccagtgtgaattctttcatgcatacttaggcatgaggaaagagcaaatgctttcccaaattctttacatacaaaaggtttctctctggtaggagttcacaggtggggtgaggaatacagaaattctttcccacatatcttgcatttacctttctccactgtgagttttcaaatgtttactacgatgggaagaagtaatgaaggtcttcccacattcaacacattcataaggcttctctcctgtgtgaattcttctatgttgagtaagcgttgaagatctattgaaggctttcccacattccttacactgatagggtttctctccagtgtgatttcgtatgtgtatagcaaggcccgtgtactgagtgaaggcttggccacattccttacattcatagggttttattccagtgtgagttcttacatgttgagtaaggtgagttgatctagtgaaggctttcccacattccgtacatttgtgtggttttattccagtgtgaatttgaatgtgaacattaaaggatgaggaatttctaaaggatcttccacattctttacattcaaaggacttctctcctttatgagtttttgcatgtgcagaaagttgagaaaaattagtgaaggatttcccacagttcttagtcttttcggatttctttccagtatgaactgctacacactgctttaagtgtgaggaagttgtgatggctctctcacattcctgaaattcacagagtttctctccaatgtggattcccatgtgattatcaaggcttgcaaaatacttaaagccttttccacattccttacatttgtagggttgtcttccattgagaatttcaagatgcacagcaaggcctggagttaaggtgaagacttttccacatggattaaatttggaaagttcttgtccaatagaggcttccttgtgcacactgatgctgtcttttccataacaattaccctcaaaagtgttccctccattctgagctctcatgtgtgtcttaaggcaaaactgttcactgaagacctctccacaattctcacagagtttccatccactgtagcttcttgtctgcatttgtatcccagtgaatatttgattcttcaaaaaaccctgctgaagtgatgaccgtttggttctaggttgtatttcccattctgaagttaagcagaaaaagaaatccacagaggccaggttcatgtagttctccagcatcacatctctgtagaggtatttctgagttgtgtccagtaaagcccactcctctggggtgaactccacagccacatcatcaaacgtcactgaatcctggtaagaatttgaccggtggtcctctaccatcgttcctatctttgtcttttcttcaaaaggacagattggttccctgggaaaaaacccatgggacatatcaaaggctgacatcctctgaagctgatggtgagatgtgcctcaatgctgtctttcttgatgccaagatcgcctcagggcagcttatgaatcacagcggggtggactccaccacaataaaggttaaacggcactgaccatgctgagccacagccggtaaagatggcggtggcacact

SEQ ID NO: 10958 - RNA, 9276 nt, Homo sapiens
  source 1..9276: mol_type = other RNA
ctgaatagctgggactacaggtgagtgccaccacacccagctaatttttgtatttttagtagagatgggggttcaccatgttgcccaaaatggtctcaatctcttggcctcgtgatccaaccatctcagcctcccaaagtgctgggtttaaaggcatgagccactgtgcctggcccagaattctttactgctaacacgagtgggcctggttctggaggatttcccagtgggtcctgaagaaccacagtttattggcttgtgggcaaaggggtatgtgtatcagttggcctttactgtgtaataaacagccacaaaaattactagctgaaaacagcagctacttaattagcagaagcctcttgaggatggacttgcaaaccaaagttgtgctggtttctactggtcaaagcaaggactggctcacataaaaaggagagagattgcaccttcagagagtaatctcaagacatctgtaatctaccacagggtgtcactgggcctctgtcaaggagcctattctttctgccaccagatctgtctaatagcttgtgtgacaatgcacttccttctgggtctctctccaagtgtagtaagtgtatatgggaatcactttattcaaacagtgtagtgcacttagttagaaagaaaaggtattaaggaagacttatatttaaaattgttatttatggtaacaacgaaaagtaacatacaaatttcaaacatcaagaataaaataaattaaaggtatgatcaatacacatcagtacaaagaggggaacacaatgaaacaaacaaaaaaaattagatgctagaaattaatccaaattattactaattaaatgtcaggcactaaatgtgcaacataaaaggattgttaattggtattattcaagtattttttctttttttttttttttttgtgacagagtttcactcttgttgcccaggctgcagtgcaatggcgtgatctcggctcactgcaacctctgcctcccgggttcaaatgattctcctgcctcagcctcccaagtagctggcattacaggcatgcaccactaggcacagctaattttgtatttttagtagagatggggtttctcagtgttggtcaggctggtctcgaactcccgacctcaggtgatcacctgccttggcctcccaaagtgctgtgattacagacatcagccactatgcccagcggtatacagattttttaaaactccagctaaagtatgtataaaaagacacatttttttaaaaagcatacagaaagactaagaagtagaggaaaatcaagctgatgtaactatataaatatctaacagaattagtggaacagaaaacatgcaagaaatagtgtagatttttcaagcgaaatatctgaaagaattcataaacctgggtactctctaccaagattaacacaagcaaagggaaagaatgcacaattaataagttattccagaatgcaaaaggagactgaagttatacaaccagcaaaaatgaaaaatataaaaagtataaatttttgctacacatttggaaataaaaacatgcctagaagaatattctcaaaatacttatgcaagccttagttgtctttttttttttttttttatgagatggagttttgctcttgtcacccaggctggagtgcagtggcaagaactcaactcactgcaaccttcgcctcccagattcaagcaattctcctgcctcagcctcccaagcggctgggattacaggcgcccgccaactcacctggctaattttattttttgaatttttagtagagacaaaagtttcaccgcattggccaggctggtctcgaactcctgacctcaggtgaccccctgccttgacctcccaaagtgctgtgattaaagccgtgaagcaccgtgcccaacctagttgtctttttttttttttttgagacggattctcgctctgtcgtcaggctggagtgcagtggtgtgatctaggctcattgaaacctccacttcaggggttcaagagattctcctgcctcagcctcctgagtagctgggattacaggggcacaataccgtgcccagctaatttttgtatttttagtaaagacggggtttcaacatgttggccaggatggtcttgatctcttgacctcatgatctgcctgcctcagcctcccaaagtggtgggattacaggcatgagccaccactcccagcctgataactgttttatttatttatttttatttttttggagatatggggtctgtgttgcccagactgatcttgaactcctggcctcaaggaatccttctgactgagcttcccagtgtgctgggattaaaagtgtgagccactatgaccagccagaagagataattttaactttttaaaatattttgcagtattggccgggcacagtggcttgtgcctgtaatcccagtactttgggagtatgaggcatgcagatcacctgaggtcaggagtttgagaccagcctggccaacttgatgaaaccgtctctactaaaaatacaaaaatcagccaggcaaggtggaggctgtctgtaatctcagctactcgggaggctgaggcaggagaaccactggaacccaggaggtggaatttgcagtaagttgagatcacaccattgcactccagcctgggcaacgagtgaaacactaactcaaaaacaaagaaacaaacaccaactcaaaaacaaagaaacaaaccaaaaaaatgaaaatatcttgtagtatttttaaatagagatgtggtttcgctatgttgcccaggctggtttgaactccttggctcaagggatctttttgcctcagcctccaaaagtgctgggattacaggcctgagccactattcccaacctagatgactcttatagattaagaatttagaaatagtaggaacatgccccactacagtatatgacagtcattatatacaaatatcattaagggacaattttttaaaaatcacaatgttattcaaacatagctccataacatattagtaaaggtcatgaagtatttttaagtgatccattatgtcacagtcgagcttatccaggaatacaaggttgatgtaacattggaaaagcaataaatacaaataccacatttatttaatttaatttatttatttttgacagagtcgcaccctgtcacccagcatggagtgcagtggtgcaatcttggctcaatgcaacctccacctcccaggttcaagtgattctcctgcttcagcctcccaagtagctgggattacaggtgcacatcaccacacccagctaatttttgtattgttagtagagatggggtttcaccatgttggctgggctggtctcgaactcttgacctcaaatgatctgcccacccccacctcccaaattgctgggattacaggcataagcccccacacccagcctgaccacatttgttttagaaaagcgcctttccatgcattcacttcttcaagttttttttttgttttgtttttgtttttttttttgagatggggtcttgctatgttgcctaagctggtctagaacccctgggctcaggccaccctcccaagtagctaaaactataggcatgcatcaccacatcatttcattgaagtatttattaggtaccatcatgagctaggtgcagttctaggtattgagttttatcagtaaataaacatgatcatcacagaggatgtgaaggaagcatttaataaattcaagaggaattcagcctcataaactatgaaatattgggaaataattcatcatgtaaaaactggatataaagaaaaaacttttcctgcaggacattgttgcaggaagtcagggaccccaaacggggggactggctgaagccatggcagaaaaacatggattgtgaaggtttcatggacatttattagttccccaaattaatacttttataatttcttatgcctgtctttactgcaatctctaaacataaattgtaaagatttcatggacacttatcacttccccagtcaatacccttgtgatttcctatgcctgtctttactttaatctctcaatcctgtcagctgaggaggatgtatattacctcaggaccctgtaataattgcattaactgcacaaattatacagcatgtgtgtttgagcaatatgaaatctgggcaccttgaaaaaagaacaggataacagcaatgtttaggaaacaagagagataaccttaaattctgaccgccggtgagccaggtggaacaaagccacatttctcttctttcacaagcaaatgggagaaatatcactgaattctttttctcagcaaggaacatccttgagaaagagaatgcacacctgggagtgggtctctgaactggcccccctgggtgtagccatctcttatggtcgagactgcaggggtgaaatagaccccagtctcccatagcactcccaggcttattaggaagaggaaattcccacctaataaattttagtcagaccagttgatctcaaaaccgtctcctgataagatgttatcaatgacaatggtgcccaaaacttcattagcaattttaatttcaccttggtcctgtgatctcgccctgcctccacttgccttgtgatattctattaccttgtaaagtacttgatgtctgtgacccacacctatttgcacactccctccccttttgaaaatccctaataaaaacttgctggtttttgcggcttgtggggcatcacggaacctaccgacatgtgatgtctgccccggacacccagctttaaaatttctctcttttgtactctgtccctttatttctcaagttggctgacacttagggaaaatagaaaagaacctatgtgaatatcggggctggttccctgacaggacataacctcttcaaaaaataaaaaagaaataaaagcctacagccaaaccaacaaaatagagtgcatatctcaccagaactgcaaagacaagtatgctggtattactacttttagttggtgttgtgcagcgggttaaaatcagtccagtaaagcaagaaaatatttagagagagcttcatcatcatacgaattttgggggtcattgttcagtccaaagtacttaatatgattcttttctctttccacatagagaatcagataatctataaataatgactcttactgttccactttaggagttaggtatacatacatatgtgtatatatatgtatatatatatacacatacacacacacacacacacacacacagtgaccccccaaatttcatatgaagttccaaacctcaatgtgactgtatgtgaaaagagaagggggcggggaggggggagaccgaccgacctatttgttggtctccatcgtgtgaaaacatgaggaagtgggcacttacatgccaggaagagagctctcactagaggttgaccatgctggcactctgatctcagacttccagcctccagatatgtgagaatataaatttgtgttttgggccagatacggtggctcaggcctgtaatcccagcactttgggaggccaaggcaggtggatcaccaaaggtcagatctgaccaacatggagatcagcctaaccaacatggagaaaccctgtctctactaaaaatacaaacttagctaaggtttgtggtgcatgccaataatcccagctactgagggtgaggcaggagaatcactggaactcaggaggtggaggttgcggtgagccaagatcataccattgcactccagcctgggcaacaagagcaaaactccatctcaaaaaaaaaaaaaaaaaaaaaaaaaaaatcctgtgtttttaacctcattgatttaaaattaaattaatttctaagccatttggtctgcggtattctcttatggttgtctgagctgactaaggcagatattggtactgagaagtgaggtactgcaattaaaaacaaacaaaaaaactaaaaatgtgaagcagctttgaaactgacaaatgagtagaggctggaaaaattctgatgtgcaagctggaaataaggttggtaagggttattctggtgaggtgtcattggggaatgaggaacatgctattgggaaatgaagaaaagacaacccttgatataaagtggtgaagaacttggcagaactgtattctagcattttacggaaggtagagcttgagacagataaaatggtatgtatcactaagatctgtaattaaagtgttaaaggacacaggaagcttcattattcctgagtgcttacaggaaaatgtgctgggaacaggccccccaaatctggccataaacaggcaatgagaaactggccataaacaaaatctctgcagcactgtgacatgctcgtgatggctatgacgcccatgctggaggctgctggtttaccagaatgagggcaagcaacacctggcccacccagggcagaaaactggaaaactgctcaaggcattcctaaaccacaaacaatagcatgagtgatttgtgccttaaggacatattcctgttgcagataacaagccagagcctgtccctttctttctcataaggaatacttatagctgatctacaatctataggaataatgtttatcacaggcttactgtcaataaatatgtgggtcaaactctgttcaagctcagctctgaaggctgtgagccccgattcccactctgcactatatttctgtgtctttgtcttaattcctctagagccactgggttagggtctccacgacccagctggtctcggcaaaaatgcaaaaggagacctgaattgcagaagaaattgttaaggaaaaaggaaccagaacttggagatttggaaaattctcagcctatccatactgcaaaaattagaaaacttgtactgaagagaatcctcaaagtgtggctgaacaatcatttgataaagagatcatgagtgggattcatggactatatcagccatcttaacagaagtgagaagagagactggattatactataagagacactgccacttacattgtgccacctaaaatggacagagaagacagaacagaacagtcaaggttgtcacacttcttattttacaagaaggggacatagaaataatcagctgtgaaagggcactggcagttatggatggtttcactcctgacatgctctgcaggatccatgggaacagaagagaaccttggaggagcatctttttaacaatccacctctggggcctacatcatcttggcttctggtaaattttgacatgaatgtgccacactggcagccactaaccaacaggggctgggatcaatctgcatgatttatctcgtacagaacttgttaatgctatgatcttaggaatctaatcaccaaggtgaggcagcctgcagtactgacctcaccatccatgacccttcttcacagatgcccagactcaggtaaccatgatgttgtattcagaacctgtaggtttaatttcagaccctcgggatgcatctaaggccaatctgtgagccattacaacctccaaaaggcatttaggactaatctgatgatctttgcactgccaataattaaagatggcaaccaatgggctaaatggtaacaacactcatatccttacattcatagtatttctccccagtgtgaattctttcatgcatacttaggcatgaggaaagagcaaatgctttcccaaattctttacatacaaaaggtttctctctggtaggagttcacaggtggggtgaggaatacagaaattctttcccacatatcttgcatttacctttctccactgtgagttttcaaatgtttactacgatgggaagaagtaatgaaggtcttcccacattcaacacattcataaggcttctctcctgtgtgaattcttctatgttgagtaagcgttgaagatctattgaaggctttcccacattccttacactgatagggtttctctccagtgtgatttcgtatgtgtatagcaaggcccgtgtactgagtgaaggcttggccacattccttacattcatagggttttattccagtgtgagttcttacatgttgagtaaggtgagttgatctagtgaaggctttcccacattccgtacatttgtgtggttttattccagtgtgaatttgaatgtgaacattaaaggatgaggaatttctaaaggatcttccacattctttacattcaaaggacttctctcctttatgagtttttgcatgtgcagaaagttgagaaaaattagtgaaggatttcccacagttcttagtcttttcggatttctttccagtatgaactgctacacactgctttaagtgtgaggaagttgtgatggctctctcacattcctgaaattcacagagtttctctccaatgtggattcccatgtgattatcaaggcttgcaaaatacttaaagccttttccacattccttacatttgtagggttgtcttccattgagaatttcaagatgcacagcaaggcctggagttaaggtgaagacttttccacatggattaaatttggaaagttcttgtccaatagaggcttccttgtgcacactgatgctgtcttttccataacaattaccctcaaaagtgttccctccattctgagctctcatgtgtgtcttaaggcaaaactgttcactgaagacctctccacaattctcacagagtttccatccactgtagcttcttgtctgcatttgtatcccagtgaatatttgattcttcaaaaaaccctgctgaagtgatgaccgtttggttctaggttgtatttcccattctgaagttaagcagaaaaagaaatccacagaggccaggttcatgtagttctccagcatcacatctctgtagaggtatttctgagttgtgtccagtaaagcccactcctctggggtgaactccacagccacatcatcaaacgtcactgaatcctggtaagaatttgaccggtggtcctctaccatcgttcctatctttgtcttttcttcaaaaggacagattggttccctgggaaaaaacccatgggacatatcaaaggctgacatcctctgaagctgatggtgagatgtgcctcaatgctgtctttcttgatgccaagatcgcctcagggcagcttatgaatctaggtggatacaggcaatctccattcccctttgtacagggttatctgaggcccacagcggggtggactccaccacaataaaggttaaacggcactgaccatgctgagccacagccggtaaagatggcggtggcacact

SEQ ID NO: 10959 - RNA, 4107 nt, Homo sapiens
  source 1..4107: mol_type = other RNA
ctgaatagctgggactacaggtgagtgtcaccatgcctggctaattttttgaatttttagtagaaacgggatcttaccatgttgcccaggctggtcttgaactcctgagctcaggcaatctgcccaccttggcctcccaaagtgctgggattacaggcacgagccaccgcacctggtctgcaagttgattcttaatatcaaagagccatggaagggttgacgttgacccccatgggtcctcagagccctttaattactttctagaccccatcaaccatctgatatcttagtgatgtcaccagtggcaaatggaacttttgatcaaatgagatccagagtgtgaccacaatacatgatgtaatcccagctccccagctatccacattagaggaaggcaagacgtcgccaatagacatactgacatattgaaaatggctttgtggacctcccctccaaaacaaacaacaacactaacaaacaaaacggaaaacctgggtgaatttctaaggacctgctacttaagaacggattaggatgaagtctctctagtccttcaaactcttacagttgatgggaatgcaccctgcatggtgttctcccaaggaacgcatctgccaggatgcacctaacggggagtaagaaagagaagggcttccttcctctctgttcccctagagtctgttctccaaagggcggccagagccaccttctaaagcctatcagaccctattgcgtttctattcaaaaccttgcgtgacttctcatttcactccgaaaaatcccaagtcttcacaatagcctgcaaaccatcccccacccctatgacctgctccccactactgccctctcccttctggcccctccctcctatggcagttgctccccatgcctggagcactctttactggacgtctacttggccacccttcccctcccttcaaatctttgtgggttgtcacctcctcactgaggcctctgtgcctccattccctgcctggtctatcttctctcccgtcgtactcatcacctaacatgctaggcgcattccttattcatgaggcctgtctcacacacgaggatgcccttcctgaagcagctctgcttccaccatgatggagtgggcacttattgtctgcagactgaacggaatgaataaggcaggtgggaggcaggggaatggctgctgggcgcttcccttcacctcactgtgcaggctctgggtgtatttccccatgaccagggggtctatgggttcttgagaagagaggatgatgtcaggggtagggtcttccaaagaaaacctgtcctgacttgcagattttatgactttcttgtcatcctttgccttgtgcttcttgctgttgggacggtcctgctctttcccgagcagcttggctcctttcttgtcttctttgtctttgatccccagttgcttcttttcctgggctgctcctttccgctcctccttcccagctttccccacaggtaccttcacttccatgataggaggtgatttttgatcttgctcttcaggcacattcaaatagatggtctccttctcaggcaggcccagcacagacctcagccacatggaatggcccaccaggctgtcaatcacatctcgccacagctgcaaacacatctggtgcaggaggttggactgcaatggccttggcttctggcacagctccagggctgctttgttgagcctcatcaacgcatcctctctgtggttctcatcagggagcaccatcactgcctttctgaagtcctccaagcagaggttccactccagcaggggaaggccatccggctcccaggggctcttggtgctgtccacatctgggctttcctccaccaggatctcctccatgatgctcttccgctgaggactcttggtccccactctggccttctgggacccggattccctgagggcctcgttctcaggccggggcacttgagtttcggagatggggctcctaaagcgtggtaacagctcagcattcacagaggccttctctgtggctatggggctgacgtgctccttgtcccctggcctggcctcctcagccttggcgggcagggtcatgtactggcgccacagttggtgcaggctttgcaccacttggtgctcataatgcagcggaggatttctgtgccggaacaagtcttcctcggtgagataggcatccacaggtgatggtgtgcgctccggggtcaagacccccatcagcagctcctgcagcacttcgcgaacgacggtgactgcctcatgggcagtcagcttgctctccagtactttcctctcatcctcaaaaacgtcctgggtcagggagaccgcgtggagattgacctgcagtatagcacctcctaatagagtaggatgggttcgaaactcccaaaattccctgaagaccccagcagtcaaagacttgaagaagaaggtaaatgttttaatttctccaggcagaatcacaccttcccggttgtcaaagtaaaatcgctgcatcctgtttttcttaaggtcttggaaagtgtccggctggtgctgccgtcgccagtcataccaaatggccacggtgccattattgaccacagtcagttctgaggaggttttctcgccttctagggtttcaaaggtcaagtgagcagcaatcccaacctgcctcttgtcctgtggattactgcctctgatccagcaagctggcttcccacagaacagcagagaagggccgagaataggcatggagacatcagaggaactggccaatgtgcctaagtatgctgtgtcttcagaggagcttccctgacttctttcaaacactgtgtagtcttccacagtaacagccgagaagggccaccctttgcccaccacctccaggccatcaatatcctgctggctgaaatccagctcttccatgattctctgcagctccttgcgtcggtagatcagaaacagactccgatcccaggtgtagcggtatgaagcgtccctctgggctggtaatcctgtctccacccggatggagtggggcttcctgatgtgagtgatgggctccatgaggccacgctgagtttttgtcttggtcatgaccagacctgtcatctcatctcccaagtattccagtcgactccagaacccactgttctcccagcttttcctatcacgccgggttggaagtgtgcagtcaatgagctcccgctcctcctggatccgtctgtaggtctccccggtgtgcatgagcagctcactcactggcttctttaggtgttcgctgagggcttcctgctgcttcttccgcagggctgtgttacgctgccagtttttcagaaagttgtgctgaggaggtggggcccagggaggtctcttctcttcttttggggctttttgctttgactctccttcagcagagatgagggtcatcagacagggtgaggtaggtatccgctcagccagctgggtgttccctcgagcaagtgcaattctcttaaaatcctggagactccccaagatgtggtggggcaggatctggtcactgccatcgaagctgtcaccgggacccatgagttgaaagacagtgaagccagggctgagactgggtgtaccggagtagtccagaggctttgtggcttcatcaggattcgcaggacgtgctacaaggtggcagaccttcctcctaggatccatgggtttgagtttacggatgataaatttctgggtgatgacacgtttatcttccttttcagtaaggcgaggaatgtgttgctccttcaagtcttccttcttaatggccaaggcaagaatgtcatctccttgtaggacattgctaacaggttcaggctcttcctgaattgtgggtgtgggttgttcaggtccctttgcccgcttcttttctttgacattctctgaggcctctaataatctggtcggagttattctgaggcgggaatccttctttagagacttcatggtgccgcccggcaccatgaaacgttgccctgcaccgccggcccagagacaccgaggctgcgccgcacccgccagccaacggccgccactgcgtccacagcaaccggtgccccgcgcgggggcgcgcatccacc

SEQ ID NO: 10960 - RNA, 2223 nt, Homo sapiens
  source 1..2223: mol_type = other RNA
ctgaatagctgggactacaggtgcaagccaccacacctgactaacttttgtattttttgtagagacaaggttttgccatgttgcccaggttggtcttgaactccagagctcaaatgatccgcccaccttggcctcccagagtgctgggattacaggtgtgagacactgcacccggcctcagaacacttcttaatggaaaacattgtcttgttgatctggaagtaatttcttttccatcagaataagccaccatacagattgaaggaaaatggtaaactcttttaacccaggggaagtccccatcttgattttgctacagcagacaatggtaccagcatcctcagagacttaggctcagaacttcagggtcatctttgacttctccctcctcatttaccactttctttagaatatccagttaaataacaaagatgctttctttgtaatgtctcccctcagccaccactggggggtcaggtacaccccacatctggcccctgtaacagcctcccaggtctcccttgccttagactctctcttctgccccaactcacacagtgctggcaggttaatcatcctcttggaacaccgttctcatcagaactttcacacgggcagtggcttctctcagataaaatcctgacacaagacataactccatccatgatttggcgtcacctctgtacagacatctcacaagtcaattttgtccacacacccctctggacacggatgccttgcaaagctgccactctgcaaggggttggctggttgccactgttgccgagtccaagctgcccgtttccgttgtaaccccagacatagacctcccccgtgtctactactgccatgcagcacatctgcccacatgctatggtcacaactactttattttgtaggcagccagtgactcttcgagggattggctgattaactgttgatccagatcctacctgcccagagttattataaccccaggcaaatacctctccatcagatgttagcaccaaagaatggtaagacccacaggcaacttcaatgacttgtttgtttgacagattagtagagatatgacagggcactaaaccatgattagttgtcccattgcccagctggctataagcattatgaccccaggtaaagacttctccttctgttgttgcaaggacaatatgtggaccactcccatagctgaggcaggctatttttttgccatttaaagaatccagtctccgaggttcaatggtgctctggacgtcacctaaccccaaacagccacagcagtttgtgccaagcacaaaaatctcatcatttactgtagtgtataaaacttcattgccagcactgccaaagacacaagcctgacgaattaactgtagttcttcttcagaacaaagggaaaaaattggccactttcccacatctaacatcttcaaagatgacagagtagcctgtactggctttgtgttggttaatgaacaagtaaatgaatggctgtgactcatttccagattcacagccctcctttccatctcatcctctgtaactccttcacacggaagccattccgaaaactgggccccaaatccctgctctcggctccaagctctccatttctacttcacctgagccatatcatcaaacacaactttgttactaagtcctcaaacttttaagtttccttctgatcacggccaacagtattaacttgtatccaaagtaaagtttgcagtcagtaaagggaagctaggatgcacggagcagctgtcccaatggccactggaccttgccactgtctccagagaaaagaggaagttcttcttccatatggactcagtcctgggcagtccctttgtcaacttttctctgggattggaaagttccaaatcacggggaagagcggacatcaattctcagctccacagaagaatatatgatttgctaagctgattgttttaaatttctggaacccagtattcagtcatctttaatcctgttccttttagatccttgtaaagttgtcttctagagcaaagttaatgtgactcctcgcaggccggagccttgtccgctccgcctcctgggtagcggttactgcacggtcaggggcccggcgccgcgatgagttggcgcctccccctgaaacggcccggcctcggcgggatgcgctcgggtgcccggccgagacggaaacgaagggagcgcagacaagaggagggggct

SEQ ID NO: 10961 - RNA, 2366 nt, Homo sapiens
  source 1..2366: mol_type = other RNA
ctgaatagctgggactacaggtgcaagccaccacacctgactaacttttgtattttttgtagagacaaggttttgccatgttgcccaggttggtcttgaactccagagctcaaatgatccgcccaccttggcctcccagagtgctgggattacaggtgtgagacactgcacccggcctcagaacacttcttaatggaaaacattgtcttgttgatctggaagtaatttcttttccatcagaataagccaccatacagattgaaggaaaatggtaaactcttttaacccaggggaagtccccatcttgattttgctacagcagacaatggtaccagcatcctcagagacttaggctcagaacttcagggtcatctttgacttctccctcctcatttaccactttctttagaatatccagttaaataacaaagatgctttctttgtaatgtctcccctcagccaccactggggggtcaggtacaccccacatctggcccctgtaacagcctcccaggtctcccttgccttagactctctcttctgccccaactcacacagtgctggcaggttaatcatcctcttggaacaccgttctcatcagaactttcacacgggcagtggcttctctcagataaaatcctgacacaagacataactccatccatgatttggcgtcacctctgtacagacatctcacaagtcaattttgtccacacaccctgtccttttccacagtgacaggagtaggataggactggttgcttttattgccagtgcccaactgcccataagaattggcgccccaagcatacacttggccttcatctgttaatactaatgtgtgtgcgtagccacaggcgaccctctggacacggatgccttgcaaagctgccactctgcaaggggttggctggttgccactgttgccgagtccaagctgcccgtttccgttgtaaccccagacatagacctcccccgtgtctactactgccatgcagcacatctgcccacatgctatggtcacaactactttattttgtaggcagccagtgactcttcgagggattggctgattaactgttgatccagatcctacctgcccagagttattataaccccaggcaaatacctctccatcagatgttagcaccaaagaatggtaagacccacaggcaacttcaatgacttgtttgtttgacagattagtagagatatgacagggcactaaaccatgattagttgtcccattgcccagctggctataagcattatgaccccaggtaaagacttctccttctgttgttgcaaggacaatatgtggaccactcccatagctgaggcaggctatttttttgccatttaaagaatccagtctccgaggttcaatggtgctctggacgtcacctaaccccaaacagccacagcagtttgtgccaagcacaaaaatctcatcatttactgtagtgtataaaacttcattgccagcactgccaaagacacaagcctgacgaattaactgtagttcttcttcagaacaaagggaaaaaattggccactttcccacatctaacatcttcaaagatgacagagtagcctgtactggctttgtgttggttaatgaacaagtaaatgaatggctgtgactcatttccagattcacagccctcctttccatctcatcctctgtaactccttcacacggaagccattccgaaaactgggccccaaatccctgctctcggctccaagctctccatttctacttcacctgagccatatcatcaaacacaactttgttactaagtcctcaaacttttaagtttccttctgatcacggccaacagtattaacttgtatccaaagtaaagtttgcagtcagtaaagggaagctaggatgcacggagcagctgtcccaatggccactggaccttgccactgtctccagagaaaagaggaagttcttcttccatatggactcagtcctgggcagtccctttgtcaacttttctctgggattggaaagttccaaatcacggggaagagcggacatcaattctcagctccacagaagaatatatgatttgctaagctgattgttttaaatttctggaacccagtattcagtcatctttaatcctgttccttttagatccttgtaaagttgtcttctagagcaaagttaatgtgactcctcgcaggccggagccttgtccgctccgcctcctgggtagcggttactgcacggtcaggggcccggcgccgcgatgagttggcgcctccccctgaaacggcccggcctcggcgggatgcgctcgggtgcccggccgagacggaaacgaagggagcgcagacaagaggagggggct

SEQ ID NO: 10962 - RNA, 2980 nt, Homo sapiens
  source 1..2980: mol_type = other RNA
ctgaatagctgggactacaggtgcaagccaccacacctggctaattttttatatttttcgtagagacggggttttgtcacgttgtgcaggctggtctcaaactcctgacctcaggtgatctgcccgcctcagcctcccaaagtgctgggattacaggtgtgagccacagtgcctggcccagactcagtttactgtaaaaatatgtaacaatttatacattttactgtgtataaaaactgtacctaaataacaggatgccaggagcagtggctcatgcttgtaatctcagtactttgggaggccaaggcaggactgcttgagctcaagagttcaagaccagcctgggtaacataggaagatcgcgtctctacaaaaaaaaaaaaaaaaattagctgggcttggtggcatgcacttgcagtcccagctgcttgggaggccaaggtgtgaggattgtttgagtctaggaggtcaaggctacagtgagccatgactgtgccactgtacttcagcctgggtgacagagtgcaaccctgtctctaaaaataaaaaaaaataataaaataaaatgcctcaggtgccaaccctgccattcattagctctatctactcactgatggaacagtgaatacatagatttgatgggggctggactacatgataaaacaactgtaacaaaatgttaacatagaacagggtggcgcatactcaggatgattcactgcacaattctttccacttctctgaaaactttcatgctggaaagaatgtccaacatgattgtttacagattgtcccaaacaatgaatgcatgaatgaatgaatacgtaaggcctcaaagatggcagaggccaggtacagtggctcacacctgtaatctcagcactttgggaggccaaggtgggcggatcacctgaggtcatgagtttgagaccagcctggccaacatggcaaaatgtcgtctgtactaaaaatataaaaattagccagacatggtagtgaccacctgtaatcccagctactcgggaggctgaggcaggagaattgcttgaaccgggaagtggaggttgcagtgagccaagatcacgccattgcactccagcctaggtgacagagtgagactctgtcaaaacaaacaaacaaacaaacaaacaaacaaaaaagggagaaatctgctgacataccttctttatgctgtctatatataggaaagtgggcatgtattactttcataataaaagtttctttttagagacaaaaacgatataagaagtccatggataaaatcggcatttattcagaaggcatgatgccaggaagaaactccccaagtgggagacaatggctggcccccctgcaagggaaacaaggcttcagcccttccctactcccagacctgccgggaaggctgggagcacagttcatggagggtctctggggtgggcctgggtgtctgacctgtccctctgcccacaggtgaatgtgacctgcgtcctgaggatcccgagtatcaggagagctggcagaggaagtcatgcagaggcaaagccaggagccccgacagggagatccccagtgtgtcagagatgcaggtggccgccattgcaaactcccggtgctcatcactggtctccagggcgatgttgtggaaggtgttcacgtaggctgcgcctcccaggagcccctcatacagaatgatcaggaagacgaggtagatgcttggcagaaagccgaaccacacgtctgccagcaggaacaccaggttgaggcactgcagcagggccagggcccaggtgaaacggatgcgacagcagcggagagaagagcgggaggcaaagacgccagcctggtacagcatctggtaccagcggtattgctgagcgtgactcagggaagtgttccagaaaaagaggagttcaaaaagtccctggttaatgaaatactcggcaaagtaaactacgaccaagggaacaatgtaccacagcagacccttgaacactgtccacctttcccgaagggagaggctggagctggagcctggcttcgactccggggcctcggttcttatgaggggctgccgggctgcgctctctgcttcttcttcccctccagggtcctgggcctcaggagatgtgagcaacaagaaatagctggccagcagcagggcagggatacccagcatggacagcagggtctgctgaggggagaggccggcctgggtgaggcccaggtaggacagggcccccagcagcccagctcccccagtccctgaggaccaccaggagatcacggccctggggtagaaggcagtgagggagaggaaggtgacctccccaaggcctgatgagatgctagcgaagaccacaccacacaggctggtccccacagaatgagaaaaggcaaccaggacgaagcttccagcagcacaaatcccactgacgagaacccgggggagccgtagagacagagttgcagtcaaatcgtgatgagctgttgtgggggatcggcgttgggcctgggtccacatggctctggtttcccgatgtcctcttgtggctaaggatgtcgtgggcggcactcagcatcaccacataagagaagttgttgcaaaggcccagcagccctcggaatccgaaaagcgccgccgcgagcctgcacagcctcccatcgcatcaagttcaggtcccccgagggtccagggtcatagagtgtccaaagggggctcccacgggagggatgagggtctgcgacaggtgacaaggatcaacgcccgattgccggtcccagctccggcttgtctagggcactcgcgccccgcgatccatcaaggaagctgggggctccatctcgagcgccctacgacccaccacgccccacccatcgtactctcccccgccccgtctacagcagggaccctgaggcctgtacctttaagagcagcagaatgttctgcactatgcagaggccgtttgtcggatcacgt

SEQ ID NO: 10963 - RNA, 3060 nt, Homo sapiens
  source 1..3060: mol_type = other RNA
ctgaatagctgggactacaggtgcaagccaccacacctggctaattttttatatttttcgtagagacggggttttgtcacgttgtgcaggctggtctcaaactcctgacctcaggtgatctgcccgcctcagcctcccaaagtgctgggattacaggtgtgagccacagtgcctggcccagactcagtttactgtaaaaatatgtaacaatttatacattttactgtgtataaaaactgtacctaaataacaggatgccaggagcagtggctcatgcttgtaatctcagtactttgggaggccaaggcaggactgcttgagctcaagagttcaagaccagcctgggtaacataggaagatcgcgtctctacaaaaaaaaaaaaaaaaattagctgggcttggtggcatgcacttgcagtcccagctgcttgggaggccaaggtgtgaggattgtttgagtctaggaggtcaaggctacagtgagccatgactgtgccactgtacttcagcctgggtgacagagtgcaaccctgtctctaaaaataaaaaaaaataataaaataaaatgcctcaggtgccaaccctgccattcattagctctatctactcactgatggaacagtgaatacatagatttgatgggggctggactacatgataaaacaactgtaacaaaatgttaacatagaacagggtggcgcatactcaggatgattcactgcacaattctttccacttctctgaaaactttcatgctggaaagaatgtccaacatgattgtttacagattgtcccaaacaatgaatgcatgaatgaatgaatacgtaaggcctcaaagatggcagaggccaggtacagtggctcacacctgtaatctcagcactttgggaggccaaggtgggcggatcacctgaggtcatgagtttgagaccagcctggccaacatggcaaaatgtcgtctgtactaaaaatataaaaattagccagacatggtagtgaccacctgtaatcccagctactcgggaggctgaggcaggagaattgcttgaaccgggaagtggaggttgcagtgagccaagatcacgccattgcactccagcctaggtgacagagtgagactctgtcaaaacaaacaaacaaacaaacaaacaaacaaaaaagggagaaatctgctgacataccttctttatgctgtctatatataggaaagtgggcatgtattactttcataataaaagtttctttttagagacaaaaacgatataagaagtccatggataaaatcggcatttattcagaaggcatgatgccaggaagaaactccccaagtgggagacaatggctggcccccctgcaagggaaacaaggcttcagcccttccctactcccagacctgccgggaaggctgggagcacagttcatggagggtctctggggtgggcctgggtgtctgacctgtccctctgcccacaggtgaatgtgacctgcgtcctgaggatcccgagtatcaggagagctggcagaggaagtcatgcagaggcaaagccaggagccccgacagggagatccccagtgtgtcagagatgcaggtggccgccattgcaaactcccggtgctcatcactggtctccagggcgatgttgtggaaggtgttcacgtaggctgcgcctcccaggagcccctcatacagaatgatcaggaagacgaggtagatgcttggcagaaagccgaaccacacgtctgccagcaggaacaccaggttgaggcactgcagcagggccagggcccaggtgaaacggatgcgacagcagcggagagaagagcgggaggcaaagacgccagcctggtacagcatctggtaccagcggtattgctgagcgtgactcagggaagtgttccagaaaaagaggagttcaaaaagtccctggttaatgaaatactcggcaaagtaaactacgaccaagggaacaatgtaccacagcagacccttgaacactgtccacctttcccgaagggagaggctggagctggagcctggcttcgactccggggcctcggttcttatgaggggctgccgggctgcgctctctgcttcttcttcccctccagggtcctgggcctcaggagatgtgagcaacaagaaatagctggccagcagcagggcagggatacccagcatggacagcagggtctgctgaggggagaggccggcctgggtgaggcccaggtaggacagggcccccagcagcccagctcccccagtccctgaggaccaccaggagatcacggccctggggtagaaggcagtgagggagaggaaggtgacctccccaaggcctgatgagatgctagcgaagaccacaccacacaggctggtccccacagaatgagaaaaggcaaccaggacgaagcttccagcagcacaaatcccactgacgagaacccgggggctgtagggcagcaggtgaaggccaagaggagccaacaatttgatgacgagtgtggggaggatgtccgccaggagcacagcagccgtagagacagagttgcagtcaaatcgtgatgagctgttgtgggggatcggcgttgggcctgggtccacatggctctggtttcccgatgtcctcttgtggctaaggatgtcgtgggcggcactcagcatcaccacataagagaagttgttgcaaaggcccagcagccctcggaatccgaaaagcgccgccgcgagcctgcacagcctcccatcgcatcaagttcaggtcccccgagggtccagggtcatagagtgtccaaagggggctcccacgggagggatgagggtctgcgacaggtgacaaggatcaacgcccgattgccggtcccagctccggcttgtctagggcactcgcgccccgcgatccatcaaggaagctgggggctccatctcgagcgccctacgacccaccacgccccacccatcgtactctcccccgccccgtctacagcagggaccctgaggcctgtacctttaagagcagcagaatgttctgcactatgcagaggccgtttgtcggatcacgt

SEQ ID NO: 10964 - RNA, 2883 nt, Homo sapiens
  source 1..2883: mol_type = other RNA
ctgaatagctgggactacaggtgcaagccaccacacctggctaattttttatatttttcgtagagacggggttttgtcacgttgtgcaggctggtctcaaactcctgacctcaggtgatctgcccgcctcagcctcccaaagtgctgggattacaggtgtgagccacagtgcctggcccagactcagtttactgtaaaaatatgtaacaatttatacattttactgtgtataaaaactgtacctaaataacaggatgccaggagcagtggctcatgcttgtaatctcagtactttgggaggccaaggcaggactgcttgagctcaagagttcaagaccagcctgggtaacataggaagatcgcgtctctacaaaaaaaaaaaaaaaaattagctgggcttggtggcatgcacttgcagtcccagctgcttgggaggccaaggtgtgaggattgtttgagtctaggaggtcaaggctacagtgagccatgactgtgccactgtacttcagcctgggtgacagagtgcaaccctgtctctaaaaataaaaaaaaataataaaataaaatgcctcaggtgccaaccctgccattcattagctctatctactcactgatggaacagtgaatacatagatttgatgggggctggactacatgataaaacaactgtaacaaaatgttaacatagaacagggtggcgcatactcaggatgattcactgcacaattctttccacttctctgaaaactttcatgctggaaagaatgtccaacatgattgtttacagattgtcccaaacaatgaatgcatgaatgaatgaatacgtaaggcctcaaagatggcagaggccaggtacagtggctcacacctgtaatctcagcactttgggaggccaaggtgggcggatcacctgaggtcatgagtttgagaccagcctggccaacatggcaaaatgtcgtctgtactaaaaatataaaaattagccagacatggtagtgaccacctgtaatcccagctactcgggaggctgaggcaggagaattgcttgaaccgggaagtggaggttgcagtgagccaagatcacgccattgcactccagcctaggtgacagagtgagactctgtcaaaacaaacaaacaaacaaacaaacaaacaaaaaagggagaaatctgctgacataccttctttatgctgtctatatataggaaagtgggcatgtattactttcataataaaagtttctttttagagacaaaaacgatataagaagtccatggataaaatcggcatttattcagaaggcatgatgccaggaagaaactccccaagtgggagacaatggctggcccccctgcaagggaaacaaggcttcagcccttccctactcccagacctgccgggaaggctgggagcacagttcatggagggtctctggggtgggcctgggtgtctgacctgtccctctgcccacaggtgaatgtgacctgcgtcctgaggatcccgagtatcaggagagctggcagaggaagtcatgcagaggcaaagccaggagccccgacagggagatccccagtgtgtcagagatgcaggtggccgccattgcaaactcccggtgctcatcactggtctccagggcgatgttgtggaaggtgttcacgtaggctgcgcctcccaggagcccctcatacagaatgatcaggaagacgaggtagatgcttggcagaaagccgaaccacacgtctgccagcaggaacaccaggttgaggcactgcagcagggccagggcccaggtgaaacggatgcgacagcagcggagagaagagcgggaggcaaagacgccagcctggtacagcatctggtaccagcggtattgctgagcgtgactcagggaagtgttccagaaaaagaggagttcaaaaagtccctggttaatgaaatactcggcaaagtaaactacgaccaagggaacaatgtaccacagcagacccttgaacactgtccacctttcccgaagggagaggctggagctggagcctggcttcgactccggggcctcggttcttatgaggggctgccgggctgcgctctctgcttcttcttcccctccagggtcctgggcctcaggagatgtgagcaacaagaaatagctggccagcagcagggcagggatacccagcatggacagcagggtctgctgaggggagaggccggcctgggtgaggcccaggtaggacagggcccccagcagcccagctcccccagtccctgaggaccaccaggagatcacggccctggggtagaaggcagtgagggagaggaaggtgacctccccaaggcctgatgagatgctagcgaagaccacaccacacaggctggtccccacagaatgagaaaaggcaaccaggacgaagcttccagcagcacaaatcccactgacgagaacccgggggctgtagggcagcaggtgaaggccaagaggagccaacaatttgatgacgagtgtggggaggatgtccgccaggagcacagcatggctctggtttcccgatgtcctcttgtggctaaggatgtcgtgggcggcactcagcatcaccacataagagaagttgttgcaaaggcccagcagccagaagcccaccgcgttcttccaatgcgcgccctgatggtccaacagagggagccggggctccgggacggtctcctccccctcggaatccgaaaagcgccgccgcgagcctgcacagcctcccatcgcatcaagttcaggtcccccgagggtccagggtcatagagtgtccaaagggggctcccacgggagggatgagggtctttaagagcagcagaatgttctgcactatgcagaggccgtttgtcggatcacgt

SEQ ID NO: 10965 - RNA, 7527 nt, Homo sapiens
  source 1..7527: mol_type = other RNA
ctgaatagctgggactacaggtgcaagccaccacctctggctaatttttgaatttttctgtagagacgggtttcaccatattacccaggctggttccgaactcctgaggtcaagccatctgcccacctcgacttcccagtgttgagattacaggcgtaagccaccatgtccagccaattcttacttgtttttatcctttttaaatgtatataaagctcatattaatctcaatgtttaattttagaagtgttttgggtctttattagaaatttggtagtgtttttgtaaccagaaatatatgccatagggacttaactcttatttatatcagttcacctatggtaaaattgatttcattatatgttgtttttcttaaactcgcagtttcccagaacctatcaacaacattgaggacttattgtattataaattatctttatatgaatataaagactttccctatttcaattgcgaatatacagatctgtgcactcaaaaataacaagcctattaggactcaaacagttatttgtatacccacgttcacagaagcattattcacaatagccaaaaagcagaagcaacccagtgtccattaatggatgaactgataaacaaaatacggtatttacatactacggcatatttggcctttaagaggaaagaaattctaatacatgctacaacatgaatgaactttgaagacattatggtaaatgaaataagaatgaatccatttagatatccagagtagtcaattcatagagactgaatgctggttaccagaggctgaggagagaggaggtaatgggtggttattgtttaatgaatacataatttcagtttgggaagatgaagagttctgtagacggatggtggtggtggttgcacaatagtatgaatatacttaatgccacagaattgaacacttaaaactggttaaagtggtgaattttacgatatgcatatttaatcacaataaaaaatgcttattaaaagatgtactagttatgaaatagcatacctcatctgtttcaaactgggtgtggctaacaatgaggtagaaaagcagcaagcaggtacagagatttataatggctgctctaggtcctatcgggtaaagggatcagcagatgtgaagtcaagagtctcctgtaagatttgactttcttggaaacatattttaatcctgggcctcctctttccaaatcacctatttcttttagtctttttgcagtgatactgtgtgttgcttctaacagaggttcagtttcacagcctttccctcaagtgtcttatcctaaaagtaaaacctagatgatctaaggtggtggttttcaacagggtgcaattttgcctcctatactcgcaacacccagggacagttggctatgtctggagacatttttgggttgtcacaactggaagtagggtggggagtggtgctaatgacatcaagtgggcataagccaattatgctgctagaaatcctacaatgcacaggataggctcccacaaacaaagacttaaccaaccccaaatactaacaatgcttggtttgagaaaccctgttctaaggtttttctaagttgcttgatttatggtagaaactgatcataagttaaaagtttcctccttttggattgcttgagcccaggagtttgaggctatggtgcattatgattatgcctgtgaatagtcactgtaatctagccactgcaatctatattaagaaacataggccgggcgcagtggctcacgcctgtaatcccagcactttgggaggccaaggcgggtggatcacgaggtcaggagatcgagaccatcctggctaacacggtgaaaccctgtctctactaaaaaaaaacaaaaaaaattagctgggcgtgctagcgggcacctgtagtcccagctactcaggaggctgaggcaggagaatggcgtgaacccgggaggcggagcttgcagtgagccgagatcgcgccactgcattccagcctgggtgacagagcaagactctgtctcaaaaaaaaaaaaaaaaaaaagaaagaaaagaaaagaaaaaagaaaaaggaaacatagtgagaccctgtttctttaaaaaaaaaaaaaaagtttcttcctcttattccttactttctcttctcatttattttgaggaaataggataagaaccagtggtaatactttaggtgaaaggaggctacttatgttatcattctcttcaccctggccgatcctaaccatgacactttatatcctgggggatggtgaaaaacagaggaggtggggtaggacttgtggtcaaattgttggggacagaggcaaaaaagaaaacagcaacaaaaaaatacaaatgaagaaattggaaggcagtgcctatgccatctgaattggataattcttcctaatggccatttggatatagatgagttggacagacataatttagaaacctatataaggaaatatcatgcattttaatgaggttataacccaaaatttaaaattcaattaaaaaattaaatcacagattttcccacaacatactaattcaacatactacttacgattacttaaaatttgcattttttctaaggagcaataacctaatgagtatgtaatactaatgtgtcagttaataagggcaattacttttgctcttattttcctgttatatgaaattaacaacatacctgctgcaatataactcatttggtacaatttaggtgtttcgagaaattcaacccactaagatcattagcgtaattcatttttatgctacacattaaaatggtgccttcttacagtcactttggaaaactgtttgacagtaaatactaaaactgaaaatatacacaccctacaacctggcaattccattcttaggtttatactcaatggaaatgtatacactcaccaaaagacatgtataagaatgttctacacagtactattcataatagctcagaattgaaaaattctcaaaagactattaatgggagaatgaataacttttggatgtaatgaaaaatggataaacaaacggaagactatacagcaatgagaatgaatgaactacaaatacatgcaacaataagaatggatctcactttggcaggttgaataacggcctccaaagatagccagcgtatgaatccctggaacctgtgaatgtcacttatatggcaaaagagattctgcagatgtgattaaattaaggatcttgagatagggggattatccctgctttatgcaggtgagccctaaacttagaggcagggaaagatctgactacagaagagaagatgatataatgacaaaagcaagctttgatcatagagaggaaggggtcacaagcccataaatacaggccgtcactggaagccaaaaaagggaagaaaacattctccctcacaacctcaataaagagccaaccctgctgatactttgatttaggcctaatgaaactgatttttggacttctgatctccaggactataaaagaataaatctgtgttgttttaagtcactaagtttgtggtagtttgttacagtggcaacaagaaactaaaatattcacaaaaatgatgaatgaaaaaaagtgtattatgtatgattacatttacataaaataaaaaacaggcaaaactaatctatgattttagaagtcaggatagtaactttcagcaagaaagaagacagtgttaagatggggaaagaggagggcttctggggtacacataatgctctgtgttttgatctgaagactagtatgtgagtttgtttaatttgtgaaaacctttatttgtgtactgttttgtgtgtgtgtggtatatgcagttttaaaaactgatgccttttaaacacttactaatctgataatctgccgaaaaagaatatataacatatattcaaggggatggaaaaatacttactgaacaataattttatttctcaagaacgctgaagattttgtttctctcttcaaaagatttaaaaaattttaactggcaaaacataatagtgactcttaaatgctaaaaaaaaaaaaaaaaaaaaaaaaaaaagaaaaaacctaaaaataaaatattgcataagtaagctttgttatgcctcgatcttaggactgtaaattataaaaatacaagtaaaaccacattttttgaaataacagtaaacaaaaacaaaaggcaggtactacataccaaatgaccaaaatgtcttttgggcctaagattcttgaaaatagtaaaaatggtaataatagaaatctctctatagaacattaaatataaaaaccatttataaaacacatcacaattttattgcttgaagaatacagcatatgaaatcacaagaatgtcaaaatgaaaagtcactaggcttcaaacgtataatacattatcagatgcagtaaaatattaacctgaactctgcatcagaaaaaaaaaaaaaggtgtggaaaatatctaagttgtttacttaagaaacagatatacttaaaatagaaagtataaggatgttacagtacaaattagaaaagccaacacgtattaacttatcgttctagactagactacctttggtacttaaactttttaaaaaacaatttcttctatctcatccaaatgcacttcatgggtatgacatccatgaagtaacttcaacttaaaacattcagcaaaattaaccttttcacttcatgggggaagtatatttaataaatgtataacaatatttcccttttactaaaactgcaaaatatgatcattaagaaacctaacagttataaaactttacttacttagctctccaattaaaattggaatcctgggagccacaatctatttttgggcttggtgaatacataagtttaaaagatttggcaactgacataggaatttaattacttaatactatcttaagtgacttttcctttctgtttccaaaatatagacattatgccatttcttcaacatcctggattcctataaacactaccatactgtatttattagaaccaaattaaagcttctctaacaagcaggtagaaactatttatgttccatatacggctgataagttataacacaacttatgtttcatatagggctgatcagttaattcatatagggctgatcagttgtaacataacttcttaagcaaaactaatcttttttttaaagctatcactcaattatggagacaataatgtcatctcaaaaggtaatgttggactctaggccatctagttgggaaaatgtaaaagtaattctaaaaacaataagtaaactataactacaagttaaattaaaaatccctctctcatagcaagcatgctcattaactttcatttctttcccccagcaaaggtttgaatattcataaacctcagttaaaccaagagaaccaatgtaattgtttcaaaagtaccacctatatatttgaataatatgagtatggatggactaggtaagtaatactatcaacaattactgaattggagtgaaagagtaaaaatcatgacagacttccaaactgggcagtctttgaaatgtcatagtggagctcaaaatgaattatgctgtaataaaactatagtttttacctctacacaaaacagaaacaaaataaaaaaacataaccaccaaatttatacaaatactattaaacatactccttcctagtttttgaatgtcttgaagtttttctaaacaagtatattgatctgagcatatatatttattgcctatatatgtactcattttaaaagacaaattcagatactacagaactgaactctttcaccaacccaatccaatgtctactgattcacacagcaccccccccttaataatttaaaattcacaagttttagtttagttaaaagggcagaggaaatgcaaatgcagatttagagctttgtagaaatttcactgtatttttataaacttgaagttatctgtaacactgtttattgatcaaacgaaggactcgctgctatctaaaatttcataaacaccattaaaaattcaaaattgatattatactgaaccttaaattttcaatagttcaaagagacagtttttacatgtatagcacacaatagatgaaacttaatagcagacatccctagaataccaatgacaagtccaccaagatgcatacaaaattacagataagcatttctttcactgtttttgttgtgcagggaaaaacatttatagaagaaatagaaactcagctggtgaatttcagatatcatcatcatcttcttcatcctgagaagatcccgcctgattagatgcactggctgaggcagcagcaagctgggcttgttgggcagcttgctgcatttgaagccattcctgttgggccaattctgcttgttgctgtctagcttttgcaaataattcttgttgctgtctcaataactcttcttcaggaatgccaaggttttccaaacgagaactggcctttcttctttttaatgctactgttttacactcttgcaagacttcttttacttcactgatgtaagagccaaatcccaaactttctagtgcttgtatgacatgctctggtgagatggtcttcttttccgatttgttacaaatctcattggcttcagaagatataaggtgaatgaattcagtgcagcagttcaccaccagctctcgagcatcgttggccacccggacattaggaagagtctctttgatcattttattgatagcagctctggggatagtgagatcatcatcgttgccagacgaggaagccatagtaccttcctgtttctcgcgccccggcttttaaaaactccccagctctggtccactactccaccgagatttctcaaaaagtcgccctcggagagtgatcccggggggtgctttgcgaagagggtgcagaaaatgaacggaggagcagctggcttgagggctgggaacactcgcgtgtgtgagagatttaggatgagtttgggaagaaagtgggggcccgaggattctagagagagcacagcccaggctgaggaggggaaagcgcggtggtccggaaatttgagcggctggggaaccaccttcgtgtctcctcagaggggcgggcgctgtcgcctaactggtccccaacggcgtcggagcagaggcaagatccaggggcactggcctcgccgcggtaccgggcgggtacccagcgggctcggctctatagagcccgaggccccgctgccgctgccgccgccgccagcagccgttgccgccgcctcggccaaaccatccttcagacacccgcgccgccgcctcacaacatgtccgccgctgccgctgccgctgccgctgctggaacggcgacggccgcctgggaactaatatggacagagccaggcacagtgggagtcgcagtggctgccgccgtggccgcgtagcccgaacgcagatcgtggaagccgaagacgcggcaacggtggtccctccagatgccagggaaggtttgcaggaagccgctcccgacaccctttgc

SEQ ID NO: 10966 - RNA, 2445 nt, Homo sapiens
  source 1..2445: mol_type = other RNA
ctgaatagctgggactacaggtgcacaacaccatacccaggtaatttttttggagataatgtctcactgttattcccaggctggtgtaaaaactcctgagctcaggcgatcctcccgtctcggcctcccaaagtgctggggatacaggtgtgagccaccatgcctggcttatgtttttttcaaaactagaaaatctccagatgttaaaaactaggcacatatttttatataacaatgaattgaaagatatttttaactgaaggataataaagagaggcatatcaaaacataagagctgcagctaaagcagaactcaagggaaaatatatcgtcctaaaatctatgtatacaaaaaagaaaacaagctgaaggatcagtgatctaaacttccatctcaagaagctgaatacgtaaatctacccaaagaaatcagaaagcatttctatgtttccaatgctaaagagaagagcaaaacccaattaaatagaaaaaaatcaatgaagctaaagcttagttctttgaaaaagtaatacaattgttaaagccctcaagcaaggttaatccatgaaaaaagagagaaaatataagctgccagtaccagcaacaagtatattttaactgtatactacatatataaaacactgagcatgaagaggaggaggaagacgggggaagaaaaacatgtgttttggagccatccagaagaactatattccagattccattctagtcaatttaatccaatatgcatttgttggaagagaatataaactactattagtttggtatgaaaggcctagaaggaaaaagcacatgaattttggagttggacagagttgagttcaaattcagtctctagcttgatactaaatgtaggacttacggtaaattattaggttggttcaaaaataattgtggttttgccattcctttcggtggcaaaacttgcaattacttttgcaccaacttaaatatataacctctctgagctcccattttctcatctaaaaaatgaaataataccaacctcacagcactgttggaagggttggggtaaagcaccaagtacgtgggtagcttatatcctacagaataattttcaccaacatgacccatgaccatgaagtttatggtttgactatctgtaggaagggtacaaaaatacatcatgcaacaaggtcattcatttggaaatgtaatgctttctgaaaaacttgagcattcacttttcttcacttgcctgttctaataagagaggtttggtgtggtgatttttcaatagaaaggatgttaccaatatataaataacataaaaggatcacatgagaattaaagtgaagtaacttaacatacaattttcattctaatcttatacaataatttttcttgactattgatagatcacaataaaggtatgctgatgatataagttattttaagactttggggaaaaaggcttccgtctctggcattgaccttattgtggaggaccctccaaaatcttcagctctgcaccagcaggtatgctgagtcatgtatgatgacataaaccacaaggagtcaaggagctaaaacaaccacagcgactggctcagatctcagatgtgcaagatgaatcctcaggatttttcacacactgaagaaacttgtcaggtctgtagatattcttgcaggaaaattgaatattccttttgcttataatcgattccagctcttttatggtgggatcctggcataagtctctggaatcttctcttccaccatgtatcacccaggcctctagtgtctgaaccttctctggttgcaaattatggacttccacactcccaaaagtgctgtttttgtcaaagattttactgcgggatccattgagcatcacatggaccacatcacaggcagcttctgcaaacctgcgggaaaccgttttccagaatactgaaacagggttgttgctgcagtcctttctccagtctgggcaagattgatagtttatttcttgttgcaaggtacggtctgagttcccaacttcattagtggctgatagtcttcttcagtaatgttgcaaggatgttttgaaataaatgcacccttgaaagcatcccatacactttggcagtctacatgtctcatctcaggatgaatttcagtgtacttgacgcatcgcgccaggacggtctcgggaaagcgcttggtggtgcccggaccgctccactgctggcgccacctcgggacgaccaccgcgagcaccacgacgaggatcaggaccaggatactgacgccaagacagagttgggctctcctagagagccggcagcagggtttgtccccggacaccgggctgaactcgcagttggccatagggctccaggcggggttggctgggcgaagatgaggccggcaggaggctaggcagcaagagagaggctggctgggttctgaaactgc

SEQ ID NO: 10967 - RNA, 2581 nt, Homo sapiens
  source 1..2581: mol_type = other RNA
ctgaatagctgggactacaggtgcacaacaccatacccaggtaatttttttggagataatgtctcactgttattcccaggctggtgtaaaaactcctgagctcaggcgatcctcccgtctcggcctcccaaagtgctggggatacaggtgtgagccaccatgcctggcttatgtttttttcaaaactagaaaatctccagatgttaaaaactaggcacatatttttatataacaatgaattgaaagatatttttaactgaaggataataaagagaggcatatcaaaacataagagctgcagctaaagcagaactcaagggaaaatatatcgtcctaaaatctatgtatacaaaaaagaaaacaagctgaaggatcagtgatctaaacttccatctcaagaagctgaatacgtaaatctacccaaagaaatcagaaagcatttctatgtttccaatgctaaagagaagagcaaaacccaattaaatagaaaaaaatcaatgaagctaaagcttagttctttgaaaaagtaatacaattgttaaagccctcaagcaaggttaatccatgaaaaaagagagaaaatataagctgccagtaccagcaacaagtatattttaactgtatactacatatataaaacactgagcatgaagaggaggaggaagacgggggaagaaaaacatgtgttttggagccatccagaagaactatattccagattccattctagtcaatttaatccaatatgcatttgttggaagagaatataaactactattagtttggtatgaaaggcctagaaggaaaaagcacatgaattttggagttggacagagttgagttcaaattcagtctctagcttgatactaaatgtaggacttacggtaaattattaggttggttcaaaaataattgtggttttgccattcctttcggtggcaaaacttgcaattacttttgcaccaacttaaatatataacctctctgagctcccattttctcatctaaaaaatgaaataataccaacctcacagcactgttggaagggttggggtaaagcaccaagtacgtgggtagcttatatcctacagaataattttcaccaacatgacccatgaccatgaagtttatggtttgactatctgtaggaagggtacaaaaatacatcatgcaacaaggtcattcatttggaaatgtaatgctttctgaaaaacttgagcattcacttttcttcacttgcctgttctaataagagaggtttggtgtggtgatttttcaatagaaaggatgttaccaatatataaataacataaaaggatcacatgagaattaaagtgaagtaacttaacatacaattttcattctaatcttatacaataatttttcttgactattgatagatcacaataaaggtatgctgatgatataagttattttaagactttggggaaaaaggcttccgtctctggcattgaccttattgtggaggaccctccaaaatcttcagctctgcaccagcaggtatgctgagtcatgtatgatgacataaaccacaaggagtcaaggagctaaaacaaccacagcgactggctcagatctcagatgtgcaagatgaatcctcaggatttttcacacactgaagaaacttgtcaggtctgtagatattcttgcaggaaaattgaatattccttttgcttataatcgattccagctcttttatggtgggatcctggcataagtctctggaatcttctcttccaccatgtatcacccaggcctctagtgtctgaaccttctctggttgcaaattatggacttccacactcccaaaagtgctgtttttgtcaaagattttactgcgggatccattgagcatcacatggaccacatcacaggcagcttctgcaaacctgcgggaaaccgttttccagaatactgaaacagggttgttgctgcagtcctttctccagtctgggcaagattgatagtttattttggaagtgttgaattcaccacaccatgtgaggtcatcagcaaggtagcctagcagcgtgtcctccagggtgaacatgtcccgctggacctgtgtgaactgatgggccagatcttttattctgctccaaagaagaatcttgttgcaaggtacggtctgagttcccaacttcattagtggctgatagtcttcttcagtaatgttgcaaggatgttttgaaataaatgcacccttgaaagcatcccatacactttggcagtctacatgtctcatctcaggatgaatttcagtgtacttgacgcatcgcgccaggacggtctcgggaaagcgcttggtggtgcccggaccgctccactgctggcgccacctcgggacgaccaccgcgagcaccacgacgaggatcaggaccaggatactgacgccaagacagagttgggctctcctagagagccggcagcagggtttgtccccggacaccgggctgaactcgcagttggccatagggctccaggcggggttggctgggcgaagatgaggccggcaggaggctaggcagcaagagagaggctggctgggttctgaaactgc

SEQ ID NO: 10968 - RNA, 5614 nt, Homo sapiens
  source 1..5614: mol_type = other RNA
ctgaatagctgggactacaggtgcacaaccacgcccggctaatttttgtatttttagtagagacggggtttcaccatgttggccaggctggtctcaactcctgaccttgtgatccacccacctcagcctcccgaagtgctgcaattacaggcgtgagccaccaggcctggctagatttatttttagaacaaggttgagtaaactctggcaagattaggtcctgacctgaattgtcacctgtgctatttcacccattgacagagaatataacatttttcttttcttttttcttttttttgagatggagtttcgctatttcactcaggctggagtggagtgaagtggcgtgatctctgctcactgcaacctgtacttcccgcattcaagcaattctcctgcctcagcctcccaagtagctgggattacaggtgcccaccaccacgctaggcaaattttgtatttttagtagagatggggtttcaccatgttggccaggctggtctcaaactcctgacctcaggtgatcctcttggacacctcagcctcccagagtgctaggattacaggcgtaagccactgtgcctcgcaacatttttcttcttaatgttcgtaggaggctaaaaagacagggaaatctttcctttaacacgttcttttaagcttttatttgtgcatgctgagcaatgtagcctgtaactattctgtggctacactgcaaaagctttcttctgacattaactctcagttccgtaactgcatgttaagcatacccctacctgggaaatatctcttctgggggaaaatcacatggtgacagcattagaagcacagacggaatagaatggcctgttgtaattcgtaatttaaggagtcattgtgtcagtgctaatagtgccaagagtccagttaaaatagcatggactctgtctgaactgcaggcagcagtgggcttgtgagtctccttgggagtatcatcagctggcactttgagggcagcttgattgaaaagagccagatctgtgtgggtgactttaataaactcaggctattcctgggctgtagaatagttacacagattaagaagagagggttgtaagaggtggcagctgaatatcaccttgggagttgaacagtaattaactttatttttaacataagaaaatgatttcatttcagaacaggaaaatgctaaggatgtagctagagagcagtaattattttactgtctcaagacaatagctagagggtaccagaaagtagtcaattaacagtctgcagtctagcctacaaagtaatcacattgaagaggtacaaaactgtggacacttaattcatccagaaaagataataagcttgtctggattgctgaagggttggcatctacataggcaggtaatatttcagagattttccacaataagaactttaggatttggtaatactactattctattgtacactttcttcaagtacattaatttgtgactttcctaaaactctgcagaagagaaaactgtctcttaggttgatttgcctaaagtcataaaacacaccccacctctcctgatttttttttttttttttttttgagacagagtctcgctctgtcgccaggctggagtgcagtggcgcaatctcagctcactgtaacctccgcctcctgggttccagtgattctcctgcctcagcctcctgagtggctgggactacgggtgcccaccacaatgcccggctattttttttctaattttagtagagacagggtttcaccatgttggccaggatggtctcgaactcctgacctcgtgatccacctgcctcggcctcctaaagtgctgggattacaggcgtaagccactgcgcccagccccacctctcctgattcttaatccaatgagtcattttcacttcaccttaatgctctggttttaatatggacatctgtctctctcttgataatccatttctgaaaatcagatattctatgtaggaatacattctatgcagaagcttattttccactattttaagtgggaaaaattttaatgtattacatgtcaatgtaaaactcaacgaattcactaagtattaataaaatacagcaaaatacctatatataacaaatatcatgttaggatgttagatgctaaaaacacttgctgctctccaaatagttaatatagtaagtaacaattgctctgtgtgcaggaatacatagcacatcccctgtgatgctctgcatattcttcaaaatgtccaccaaggattctgatattctgtcaaaaatgttactcaagacatttcctgcatatcataatgttgtattgcattttggggatgtatagcttttcctatataagcaactacagtaaaacattgtatgaattttggatattaaaaaccaaaaggcagcagggtgcagtggctcacgcctataatcctaagcacattaggaggccaaggtgggcagatcacgaggtcagatcaagaccatcctggccaacatggtgaaaccctgtctctactaaaatacaaaaaattagctgggcacggtggcatgcgcctgtagtaccagctactcgagaggttgaggcaggggaatcacttgaatctgggaggcggaggttgcagtgagctgatcacgccactgcactcccgcctggcaacagagcaagactccgtctcaaaaaaaaaaaaaaaacaaaaaaaaccaaaaaaacaaaaccaaccaaaaggcttccacagggaaataactagagaggtggtcttgcagggtctgctgtaattaactggcactatgccaaggaaacaaagctaatgccagtgaaaaatacagtcatttaattctccattttgggtcaatgcaaatgcgtatctcaaaaaaaccaaggttctgaacctctggcaacatcttataattcagtaagatctgctgctggctaaacttagggcatgctagagcagagttgctgggaaaactaagagtaacatcgaactacttgcacatactgagggtacctcaaggcgctggcttccttggagtgcttggacctttaacagaaggtcttagtctaccattgtgtgtgtgcagaaggctgatttgagtttttgcatgattgcacattcatgcacgtagcattactatccatgtgtagcgagactactagatgctagtctgagtctttacctttccatcatctactgtcatgctttcccaagtctgaagatcctgttttccaagatctgtgctcagtaaacaagctttggagtctttaaatgtaaggaataggaaaggtgaagagaggcctggcttaaaatcataacatggagattatggcagtgaatcccattggattgaatggtctgatatggaaagcaggctgtgtagttccactagtccaaaaattctattttttgagacacagtctcgctctgtcacccaggctggagtgaagtggcatgatgtcgactcactgcaacctccgccttccagattcaagcgattctcctgcctcagcttcccaagtagcttggattacagacgcctgccaccacacctggctaatttttgtatttttagtagaaatggggttttgccatgttggccaggctggcctcaaactcctgacctcaagtgatccacccacctcagcctcctaaagtgctgggattacaggtgtgagccactatacctggcctggtccattctttttttttttttttttttttttaagaacaaaactagtttatttggattggggactctgaacagttctgtctctattacccgacttcctcctcccacgacttcggcacctagaggaactttggctccggctgcggtggctcctgcggctctggctccggcggccctggtcccagctgcggtgcctatttcttcctctgcttggtgaattgtgcctctcccgactctttgatgtgcgtttgtgagatttcttccccctatgactactcttttttctctcggattccccatttcttttgtaggtgtggtctggactagggtttctccttccccgctgcctgctgtagtagtggtcgtggtggcccatcttctccctcctctcggagttcttgccaaaggaggagccagtctgatctgaagacaagtagatgtctctattagcttcccagaattcattgttgggatttctgaacacatgaagaaagttgcagtgttttcctcttggacattgttgtatttcaaataaaccacaaatcgccattttccaccgggtcactgggcagaattcacattgcagctgtcgtcctgcataccatcgtccgttaaacagagaaagggctgcttggcattcttcttccgactggtactgaacatatacattgcccctcaggtgaggttccaaattgcagctgaccttgaactgaatcactttccccacgttcttgaactcgggcaacacatcctcatagaaatctaggaactgttggtaggtttcttcctcgctgtactccaggcttgcgtcagggtcatagtcatccctcctgcactgctccattccaaacgttgtaaacatgctcttaataagaagggtaggactagatgttgggaaattatgtttacgtgaacatctgtctccaaatctgcaagctcctgttttactgtagaagggacaattagctcgatccttctccattactctgaaatccacgggtggttctgggttttgccatgtggtactattttctaaatcattttcagcctgatccagcatcttctgcacagcttcctctttttctttcttctcctgttgtttctgctcctcctcttctctctctttcctctgctgttctttccattgttcctttaactttctctcttgttcttctagccattttttagccgcctcttccttttccttctttattctgaattcttcttgtgccttctgctccctcagcaaccactcctcatgtaatctttccctctctctttccaatagcttctcttcttctagttgttgttcttcaataaaagtgtcctcttcctcctcctgtgagagtcctgagtctctcagtcgagcaagttcctgccgacgtttctttcgtttctccttcttcagggcggccctgtactttttgtggcttggtttctctggaaatgtcatcttcttgggaaacgtcatcttctcaagtgcagccatcttgccagcaccgcctgacccctcagacattcttaacgtgatgggaactgtacaaggcagaggctcccatcttcctgtttgagctggacccggactctgcctctgtattggacatcacgattccattctctagagtacattttatttttctcaagaaatacgttaagtccaactgctgaacatacatcttgaatctctgtagctgtaggattttcaacagccttacttatggggattcgccttccctctgcgatggtcttcttattatttaaataagcaggatagatacaaataaacctgtcctggtcggccggggaccgcgcggcagcgcaagccatcttcacaagagtctcaacaacccaggagccgcagggagaaacccggcagaaacccgggaggaacccggctctgagtttccgagacagccc

SEQ ID NO: 10969 - RNA, 2291 nt, Homo sapiens
  source 1..2291: mol_type = other RNA
ctgaatagctgggactacaggtgcacaaccacgcccggctaattttttgtatttttagtagagacagggtttcaccgtgttagccaggatggtctcgatctcctgacctcgtgattcacctgccttggcctcccaaagtgctgggattacaggcatgagccaccatgcctggcccagattctttttgataaaggatatttctgagtggatctcctgaatggatctatctgggagtgccttgagcaaaatcactgctataggtacgtcaactagttatgtcccttataattaatacaattattaattcatacagagtataagtcaaaatcttataaaattggttaatattggttatcattcagcaaatatttattgagtatctactgtatggcaggctgggctacaggcgggggatgtaatagtgaaaaaggcagaaatggtcctttaattgccgtctgatgatgattataggcctaagtgacccgcgctcaactgatgcgacctaattcctgagcctgttaaactgcagggtaaatcatgggctgaacagtcactcagtgaagtcttatctgaaatagccaggcagtttgcccctccattataacccttagattgcctgcttttgctcttcctccttcagcaacttcatcagctcttccagctggaccatcagctcccgcctgctctcctgcagggccgacatcctctgctccagttcatccttcctttgcctcagcagccgcagctctgccagcagcgtggggttctgctgtgccttctcaggggtgggctgggaggcctgctcgtgttccaggcggagacgctgaatctcctgcaggatctctctgtttttgttttccagttctgcaataagctgtctttgttgtttgttggcatcaaagttaaagctcaagtcagtgggaggacgagtcacgtttcctgcttctgcagccagccgggcagcatagcgagctataagacggtgttcctcatccagtcggctaggactgtccagaacactcttggtgggagtgggcactccagaggacatgtggctaaccatggtgtcattcatattagtcagagggcgaggaggaactatatgtgcaaggtcaagtggtttctctggttgctcaggaaaaacaggatgcgggggttctctcgtgggtacacaccccaaagatttactaattgcatggctcagcttctttgcaggagatttccaagaggaatgctccttcatctggtgctggttgctgtgagggccgccggcatggccacgccaaaagcaattctggcagagctgatagttgtggcactgctggcatcggtaccggaaacccatcatactctcacatcggcagtaggagcactccacgggatggaagacattctcaacatgggcaagcctgtgcatgagaggtagccagacaaggcactggggaggagggtcagccatcattgtgtctaaaaacatatttagcattatctttctctgctgtggaaaacaggtgcggactgagtgctctgtgtaaccaaaagatggcccttcaaagacagctgttgggagcttcagaacttccttcagaaactggtcaaacttgctaaatatcattaagccattggaatctgacatctgggagaaaacatatctcaatttgtccagcatttttccaccacacatggttgctaacatagctttaactgaaaataccgtcaacttgcctcggccctcactgtcatatgcagcaatcataaagttgaggaggaggctgatagattgttccacactaatttggtgagtagaaggaaggcgcttgttcaactgatagtagatggaggagatgacagtttcgaggcgggacacactgatctcggtggtatggtccagtgtattaaggccattgtctcggaaggcttcaatcatgttccagatatcaacaagatgaaggttgcatcgtttttgtacaaatcgtaatttgcaggctgttctgtaagttgatagtcgtatgacatcaaaattctgagcacgcatttctatgaacagctgcctcttctctgccatggtcttccgcttgttcccactttcctcaatcatccttgctcacttccccgccggagcaggggtcgtcgggaaggtctcctgcggcctcactcctccgcacgctccggcccagccccctcggctgaggcagcggcagcgcctactcaggccccggagccacccccgcggcgaacgttcgcagcgcccggctcgcgccgcttctccgcccggcacgcgcagcgcccgc

SEQ ID NO: 10970 - RNA, 8537 nt, Homo sapiens
  source 1..8537: mol_type = other RNA
ctgaatagctgggactacaggtgcacaccaccaagcctggctaattttttgtattttagcacagatgaggtttcactatgttggccgggatggtctctatctcctgacctcgtgatccacccgcctcggcctcccaaagtgctgggattacaggcgtaagccaccacacccggcctgtaatttcattataacattgatgaaaaacaattatttacaaccagggccactgtctgtgtgaattttgcatgtcctccacatatctgcatgagttttctctgggtattctggtttcttctcaattcccaaagatgcacgttaggtgaattggtacagctaaatggtcccagtatgcgtgtgtgtgccgtgtgagtgcgccctgtgatgaaaaggcatcctgtccagggttggctcccactttgctccctgagctgctgggataggctccagctacccaagacactgaactgaaataagcaggttgaaaaacgaatgaatacaaattactgtaaaacgaaaatttgtaaagtatataataatcatacaaatgcacaataaatgatgcagtatgaaagcactcagcaagcccactttatttcttattttttgtttttgaactgcatggtggtaggaggtgctccttaaaattttcacttcccaacagttattccttgatttaacccactagcactacaactgctgtcactcactgattcgccaaatattgggtaaataatttttactttttttttttttttttgagacagggtctcattctgtcacccaggctggaatgcagtggtaccatcacggctcaccgcagcaccgactgtgggattgtttaatgcagggtttatcaataacaaccccataaacatttggggctggataatatatatattttttttgagataggattttgctctgttgcccagactggagtgcagtagcgtgatcatggctcactgcagcctcgacctcccaggctcaagggatcctcccacatcaggctcccgagtagctgggactacaggtgcaagccaccacctctggctaatttttgaatttttctgtagagacgggtttcaccatattacccaggctggttccgaactcctgaggtcaagccatctgcccacctcgacttcccagtgttgagattacaggcgtaagccaccatgtccagccaattcttacttgtttttatcctttttaaatgtatataaagctcatattaatctcaatgtttaattttagaagtgttttgggtctttattagaaatttggtagtgtttttgtaaccagaaatatatgccatagggacttaactcttatttatatcagttcacctatggtaaaattgatttcattatatgttgtttttcttaaactcgcagtttcccagaacctatcaacaacattgaggacttattgtattataaattatctttatatgaatataaagactttccctatttcaattgcgaatatacagatctgtgcactcaaaaataacaagcctattaggactcaaacagttatttgtatacccacgttcacagaagcattattcacaatagccaaaaagcagaagcaacccagtgtccattaatggatgaactgataaacaaaatacggtatttacatactacggcatatttggcctttaagaggaaagaaattctaatacatgctacaacatgaatgaactttgaagacattatggtaaatgaaataagaatgaatccatttagatatccagagtagtcaattcatagagactgaatgctggttaccagaggctgaggagagaggaggtaatgggtggttattgtttaatgaatacataatttcagtttgggaagatgaagagttctgtagacggatggtggtggtggttgcacaatagtatgaatatacttaatgccacagaattgaacacttaaaactggttaaagtggtgaattttacgatatgcatatttaatcacaataaaaaatgcttattaaaagatgtactagttatgaaatagcatacctcatctgtttcaaactgggtgtggctaacaatgaggtagaaaagcagcaagcaggtacagagatttataatggctgctctaggtcctatcgggtaaagggatcagcagatgtgaagtcaagagtctcctgtaagatttgactttcttggaaacatattttaatcctgggcctcctctttccaaatcacctatttcttttagtctttttgcagtgatactgtgtgttgcttctaacagaggttcagtttcacagcctttccctcaagtgtcttatcctaaaagtaaaacctagatgatctaaggtggtggttttcaacagggtgcaattttgcctcctatactcgcaacacccagggacagttggctatgtctggagacatttttgggttgtcacaactggaagtagggtggggagtggtgctaatgacatcaagtgggcataagccaattatgctgctagaaatcctacaatgcacaggataggctcccacaaacaaagacttaaccaaccccaaatactaacaatgcttggtttgagaaaccctgttctaaggtttttctaagttgcttgatttatggtagaaactgatcataagttaaaagtttcctccttttggattgcttgagcccaggagtttgaggctatggtgcattatgattatgcctgtgaatagtcactgtaatctagccactgcaatctatattaagaaacataggccgggcgcagtggctcacgcctgtaatcccagcactttgggaggccaaggcgggtggatcacgaggtcaggagatcgagaccatcctggctaacacggtgaaaccctgtctctactaaaaaaaaacaaaaaaaattagctgggcgtgctagcgggcacctgtagtcccagctactcaggaggctgaggcaggagaatggcgtgaacccgggaggcggagcttgcagtgagccgagatcgcgccactgcattccagcctgggtgacagagcaagactctgtctcaaaaaaaaaaaaaaaaaaaagaaagaaaagaaaagaaaaaagaaaaaggaaacatagtgagaccctgtttctttaaaaaaaaaaaaaaagtttcttcctcttattccttactttctcttctcatttattttgaggaaataggataagaaccagtggtaatactttaggtgaaaggaggctacttatgttatcattctcttcaccctggccgatcctaaccatgacactttatatcctgggggatggtgaaaaacagaggaggtggggtaggacttgtggtcaaattgttggggacagaggcaaaaaagaaaacagcaacaaaaaaatacaaatgaagaaattggaaggcagtgcctatgccatctgaattggataattcttcctaatggccatttggatatagatgagttggacagacataatttagaaacctatataaggaaatatcatgcattttaatgaggttataacccaaaatttaaaattcaattaaaaaattaaatcacagattttcccacaacatactaattcaacatactacttacgattacttaaaatttgcattttttctaaggagcaataacctaatgagtatgtaatactaatgtgtcagttaataagggcaattacttttgctcttattttcctgttatatgaaattaacaacatacctgctgcaatataactcatttggtacaatttaggtgtttcgagaaattcaacccactaagatcattagcgtaattcatttttatgctacacattaaaatggtgccttcttacagtcactttggaaaactgtttgacagtaaatactaaaactgaaaatatacacaccctacaacctggcaattccattcttaggtttatactcaatggaaatgtatacactcaccaaaagacatgtataagaatgttctacacagtactattcataatagctcagaattgaaaaattctcaaaagactattaatgggagaatgaataacttttggatgtaatgaaaaatggataaacaaacggaagactatacagcaatgagaatgaatgaactacaaatacatgcaacaataagaatggatctcactttggcaggttgaataacggcctccaaagatagccagcgtatgaatccctggaacctgtgaatgtcacttatatggcaaaagagattctgcagatgtgattaaattaaggatcttgagatagggggattatccctgctttatgcaggtgagccctaaacttagaggcagggaaagatctgactacagaagagaagatgatataatgacaaaagcaagctttgatcatagagaggaaggggtcacaagcccataaatacaggccgtcactggaagccaaaaaagggaagaaaacattctccctcacaacctcaataaagagccaaccctgctgatactttgatttaggcctaatgaaactgatttttggacttctgatctccaggactataaaagaataaatctgtgttgttttaagtcactaagtttgtggtagtttgttacagtggcaacaagaaactaaaatattcacaaaaatgatgaatgaaaaaaagtgtattatgtatgattacatttacataaaataaaaaacaggcaaaactaatctatgattttagaagtcaggatagtaactttcagcaagaaagaagacagtgttaagatggggaaagaggagggcttctggggtacacataatgctctgtgttttgatctgaagactagtatgtgagtttgtttaatttgtgaaaacctttatttgtgtactgttttgtgtgtgtgtggtatatgcagttttaaaaactgatgccttttaaacacttactaatctgataatctgccgaaaaagaatatataacatatattcaaggggatggaaaaatacttactgaacaataattttatttctcaagaacgctgaagattttgtttctctcttcaaaagatttaaaaaattttaactggcaaaacataatagtgactcttaaatgctaaaaaaaaaaaaaaaaaaaaaaaaaaaagaaaaaacctaaaaataaaatattgcataagtaagctttgttatgcctcgatcttaggactgtaaattataaaaatacaagtaaaaccacattttttgaaataacagtaaacaaaaacaaaaggcaggtactacataccaaatgaccaaaatgtcttttgggcctaagattcttgaaaatagtaaaaatggtaataatagaaatctctctatagaacattaaatataaaaaccatttataaaacacatcacaattttattgcttgaagaatacagcatatgaaatcacaagaatgtcaaaatgaaaagtcactaggcttcaaacgtataatacattatcagatgcagtaaaatattaacctgaactctgcatcagaaaaaaaaaaaaaggtgtggaaaatatctaagttgtttacttaagaaacagatatacttaaaatagaaagtataaggatgttacagtacaaattagaaaagccaacacgtattaacttatcgttctagactagactacctttggtacttaaactttttaaaaaacaatttcttctatctcatccaaatgcacttcatgggtatgacatccatgaagtaacttcaacttaaaacattcagcaaaattaaccttttcacttcatgggggaagtatatttaataaatgtataacaatatttcccttttactaaaactgcaaaatatgatcattaagaaacctaacagttataaaactttacttacttagctctccaattaaaattggaatcctgggagccacaatctatttttgggcttggtgaatacataagtttaaaagatttggcaactgacataggaatttaattacttaatactatcttaagtgacttttcctttctgtttccaaaatatagacattatgccatttcttcaacatcctggattcctataaacactaccatactgtatttattagaaccaaattaaagcttctctaacaagcaggtagaaactatttatgttccatatacggctgataagttataacacaacttatgtttcatatagggctgatcagttaattcatatagggctgatcagttgtaacataacttcttaagcaaaactaatcttttttttaaagctatcactcaattatggagacaataatgtcatctcaaaaggtaatgttggactctaggccatctagttgggaaaatgtaaaagtaattctaaaaacaataagtaaactataactacaagttaaattaaaaatccctctctcatagcaagcatgctcattaactttcatttctttcccccagcaaaggtttgaatattcataaacctcagttaaaccaagagaaccaatgtaattgtttcaaaagtaccacctatatatttgaataatatgagtatggatggactaggtaagtaatactatcaacaattactgaattggagtgaaagagtaaaaatcatgacagacttccaaactgggcagtctttgaaatgtcatagtggagctcaaaatgaattatgctgtaataaaactatagtttttacctctacacaaaacagaaacaaaataaaaaaacataaccaccaaatttatacaaatactattaaacatactccttcctagtttttgaatgtcttgaagtttttctaaacaagtatattgatctgagcatatatatttattgcctatatatgtactcattttaaaagacaaattcagatactacagaactgaactctttcaccaacccaatccaatgtctactgattcacacagcaccccccccttaataatttaaaattcacaagttttagtttagttaaaagggcagaggaaatgcaaatgcagatttagagctttgtagaaatttcactgtatttttataaacttgaagttatctgtaacactgtttattgatcaaacgaaggactcgctgctatctaaaatttcataaacaccattaaaaattcaaaattgatattatactgaaccttaaattttcaatagttcaaagagacagtttttacatgtatagcacacaatagatgaaacttaatagcagacatccctagaataccaatgacaagtccaccaagatgcatacaaaattacagataagcatttctttcactgtttttgttgtgcagggaaaaacatttatagaagaaatagaaactcagctggtgaatttcagatatcatcatcatcttcttcatcctgagaagatcccgcctgattagatgcactggctgaggcagcagcaagctgggcttgttgggcagcttgctgcatttgaagccattcctgttgggccaattctgcttgttgctgtctagcttttgcaaataattcttgttgctgtctcaataactcttcttcaggaatgccaaggttttccaaacgagaactggcctttcttctttttaatgctactgttttacactcttgcaagacttcttttacttcactgatgtaagagccaaatcccaaactttctagtgcttgtatgacatgctctggtgagatggtcttcttttccgatttgttacaaatctcattggcttcagaagatataaggtgaatgaattcagtgcagcagttcaccaccagctctcgagcatcgttggccacccggacattaggaagagtctctttgatcattttattgatagcagctctggggatagtgagatcatcatcgttgccagacgaggaagccatagtaccttcctgtttctcgcgccccggcttttaaaaactccccagctctggtccactactccaccgagatttctcaaaaagtcgccctcggagagtgatcccggggggtgctttgcgaagagggtgcagaaaatgaacggaggagcagctggcttgagggctgggaacactcgcgtgtgtgagagatttaggatgagtttgggaagaaagtgggggcccgaggattctagagagagcacagcccaggctgaggaggggaaagcgcggtggtccggaaatttgagcggctggggaaccaccttcgtgtctcctcagaggggcgggcgctgtcgcctaactggtccccaacggcgtcggagcagaggcaagatccaggggcactggcctcgccgcggtaccgggcgggtacccagcgggctcggctctatagagcccgaggccccgctgccgctgccgccgccgccagcagccgttgccgccgcctcggccaaaccatccttcagacacccgcgccgccgcctcacaacatgtccgccgctgccgctgccgctgccgctgctggaacggcgacggccgcctgggaactaatatggacagagccaggcacagtgggagtcgcagtggctgccgccgtggccgcgtagcccgaacgcagatcgtggaagccgaagacgcggcaacggtggtccctccagatgccagggaaggtttgcaggaagccgctcccgacaccctttgc

SEQ ID NO: 10971 - RNA, 3045 nt, Homo sapiens
  source 1..3045: mol_type = other RNA
ctgaatagctgggactacaggtgcacaccaccacacccagcaaatttttgtatttttaatagagacggcatttcaccatgttggtctcgaactcctgacctcatgatctgcctgctttggcctcccaaagtgctgggattacaggcgtgagccactgcactcagccacatgtggatttctttatgcgtggagtgcttctgccttgaaggcagtcagagccttccttagacccaggtgtcgtagtaactgtcatgcaggcctaggaaccccaactgccccggtgttccccagtgtggcccgcttggctcccccagccctcctgccgccctcatcctttcttctgtggtggctggaggcccccggggtctgatggagctgctcttggccacctgcaggttctcttctgctttgagcagtttgatgagctcaccctgctgcaccttcgtgagtttgacaagaagaagctgatctctgtggagacggacatagtcgtggatcactacaaggaggagaagtttgaggacaggtccccaggtcggcatcccctgctctctaggcgtggggctggtttccactccccgcacgcctctcctgccccgcagcgagggcttcctttgggttttcgtcagttgacctgggctcagccacccccgagaagagccttgtgggagcaccctggtgactggaggaaggtgcctcctggtttagatatcaggggtctgtccagtgctcctgccacggtggcttctggagctggcccagcttcttgagaggctgtgtatttttttaaagccctaaccaagttgtatgggcctcaggcaacctgaagcatcctttgaggttttacttttagatgaaaagcatcttgctagcttgtgtctccatcctggtgggagaggaggtgggagctggaagcatgctgcgtggcccccatggaagccggggagttgggatgcaggcctgagctccctgtcgcctgctcttccgcagccgccgagtgcctatcagagaaggagacggaggagctcatggcctggatgagaaatgtgctggggtcgcgtgtcaccaacgtgaaggtgaggctttcccggggatggaccaccacttggccgcagtgtccctaacaggctggccagctggtggctcccagtacctggcccgttgggtgtccttccagcagcagcagaagcccttggtgtcaggtggagaccctgtgggtccctgctcggcacgtgttgctcgggagtgccgctgaggcaggaaggccgtgtctttctcccagccctgctccagagcaggtgtgaactgagaacagttggtcactcaggccataggcagcctggaagttaaagggaagagccgagtcgggaacaacggcgcctcggagcagcatccctgcaaccacgatcctgtcataggcacagtgcgtgggtgtagctgtggtgtcagcgctgtcggggatcagccactggaaggtggggcttgtccacaggcggatggatgaccactgggagggtctcacatagctgcagcccgcattgaagtcgcccatcaacatgacgtcctccaagccccatttctcttggacatccaggtagacgtcatagagagcgtcgatctcggctactgcgtcccccggggccgcatgcaggggaacaatggcaaactccctgacctctgtgaaccgggagaagaacctgacaatggctggctctcggttgaaggtgtcgttcccgcagggctcgcagccatcatcgtagtagtagctgtccaccgcagacacctggtcaggcctgtacacgaacaggtagcgctccttatagctgttccgtcccagtggctcactgaccacgtagtgataggtgtctggtgcatccctgcacaatgtagctgacgagggtggcattggacatcttggtctccccaaatgtctggatgttgaaggctgcgatcttcagggacacggccccctgcagtagggccgccagtgccagcagcgcccccagcagcttcatgcccctcatcctgagatgatggtgatgtcctcagagatgacgagaatgctgtcaagaatctggaatatcctttgatgacaattttctccttttgctccccaagcttccctgtgttgtgctgctgggcggctctccaggccttcaagctggggccttctgaacggtggccggctcctcgggtcctgggcaggagtgcttccccgtgagctcttccacaccagacgcagagcctgcggaaccttgccaaggcggcttcctaagctcctcccctgtggcccacatggaggggtggctgctggtcagggccacgccccccacagcgtggagctgcagcagggccatgctggccaccactagccaccctgccacagctgcagctgtggatggggcctcacgcaggagcagcaacagcacctgggggctggggatgagtctagcttggtgctgatccacccaaatccagagtgaccacatccgagtggccctgttgggcctgctccccactgtccaaagtccactggagtcacggtggagccatcgagacaggacagtggctctgcccttgagagctcatgggtgacgggctcctgtcctcgcttgagcccatgaggaggtgctgatcttcggaggtgcctgggcccaggagtgacagccacaggaagctagtgacatgcaacttgctggggaggccactacccaggctggcgctgtaccactcagcaagcttttgccatcttgctgttcccattcatattgtggtcactgagaggaagcttctcgggcccccaggccagatttggtgcctctcccggtccccctcacaccgtccactctccgctccacaggcaggtatgcccagagggggccgccgttgtatccgcgaacatttcctgagccagctggggaggaaccagactttatctcacagctgccacagtgccttaaactcgccctaactctttctcaaaaactaacagactccacctgaagcaagcgccgcttccgcctcgccccgcctcctgccgaccgg

SEQ ID NO: 10972 - RNA, 3240 nt, Homo sapiens
  source 1..3240: mol_type = other RNA
ctgaatagctgggactacaggtgcacaccaccacacccagcaaatttttgtatttttaatagagacggcatttcaccatgttggtctcgaactcctgacctcatgatctgcctgctttggcctcccaaagtgctgggattacaggcgtgagccactgcactcagccacatgtggatttctttatgcgtggagtgcttctgccttgaaggcagtcagagccttccttagacccaggtgtcgtagtaactgtcatgcaggcctaggaaccccaactgccccggtgttccccagtgtggcccgcttggctcccccagccctcctgccgccctcatcctttcttctgtggtggctggaggcccccggggtctgatggagctgctcttggccacctgcaggttctcttctgctttgagcagtttgatgagctcaccctgctgcaccttcgtgagtttgacaagaagaagctgatctctgtggagacggacatagtcgtggatcactacaaggaggagaagtttgaggacaggtccccaggtcggcatcccctgctctctaggcgtggggctggtttccactccccgcacgcctctcctgccccgcagcgagggcttcctttgggttttcgtcagttgacctgggctcagccacccccgagaagagccttgtgggagcaccctggtgactggaggaaggtgcctcctggtttagatatcaggggtctgtccagtgctcctgccacggtggcttctggagctggcccagcttcttgagaggctgtgtatttttttaaagccctaaccaagttgtatgggcctcaggcaacctgaagcatcctttgaggttttacttttagatgaaaagcatcttgctagcttgtgtctccatcctggtgggagaggaggtgggagctggaagcatgctgcgtggcccccatggaagccggggagttgggatgcaggcctgagctccctgtcgcctgctcttccgcagccgccgagtgcctatcagagaaggagacggaggagctcatggcctggatgagaaatgtgctggggtcgcgtgtcaccaacgtgaaggtgaggctttcccggggatggaccaccacttggccgcagtgtccctaacaggctggccagctggtggctcccagtacctggcccgttgggtgtccttccagcagcagcagaagcccttggtgtcaggtggagaccctgtgggtccctgctcggcacgtgttgctcgggagtgccgctgaggcaggaaggccgtgtctttctcccagccctgctccagagcaggtgtgaactgagaacagttggtcactcaggccataggcagcctggaagttaaagggaagagccgagtcgggaacaacggcgcctcggagcagcatccctgcaaccacgatcctgtcataggcacagtgcgtgggtgtagctgtggtgtcagcgctgtcggggatcagccactggaaggtggggcttgtccacaggcggatggatgaccactgggagggtctcacatagctgcagcccgcattgaagtcgcccatcaacatgacgtcctccaagccccatttctcttggacatccaggtagacgtcatagagagcgtcgatctcggctactgcgtcccccggggccgcatgcaggggaacaatggcaaactccctgacctctgtgaaccgggagaagaacctgacaatggctggctctcggttgaaggtgtcgttcccgcagggctcgcagccatcatcgtagtagtagctgtccaccgcagacacctggtcaggcctgtacacgaacaggtagcgctccttatagctgttccgtcccagtggctcactgaccacgtagtgataggtgtctggtgcatccctgcacaatgtagctgacgagggtggcattggacatcttggtctccccaaatgtctggatgttgaaggctgcgatcttcagggacacggccccctgcagtagggccgccagtgccagcagcgcccccagcagcttcatgcccctcatcctgagatgatggtgatgtcctcagagatgacgagaatgctgtcaagaatctggaatatcctttgatgacaattttctccttttgctgcttaaagaaaaaaaagtagtctatgaagaaaggtctctgaagaagcacttcaaggccctggcagtgctgctgggctccggatcctgcacaggcagtgcgtgtctgggagttttaaaagttcaggcagctgtgaccttccctggggcaaatgtgagccgtcacctgagagtgcagaaaacaatggctctgtgtggctttccgcataggtgggttgctagcacgtgtttctttctgtaagcacaggtttcttgctgctgtaaaaactgcacctgataatcacgtttgcacttagttttaaaatgtctgataacaaggccaaaggttcctatcccgtgtcccttgcacgtgtggtggcccccatcttccaggatagggcagggatgggccaggtatgtgcgggagggtggggctgggctccagtctccctgtctcttgtctgggggccccaaggtcactttggacaaagaggccaaagccacatccaaagttgcaaatggagccccctggtggctgacagccatgactgctctgtggcccaggacacgcctgccttcctgattcatcgccatcaggtgcaggcaactctgcaggaggctggggagctcggaacaagcagtggtgggggcctgcagcaccagcgccgtggggccaggacaggtggggcctgcaaagcccaccccaattgccagccaagcagtggggagccttcttgaggtagacaataggctgtgtgtttaggcccaggggatcccgagtgaccaggtcacaagggcagggcagcagctaaaggccaggcctcaggtccagtaatttcttggttcttttgttttgggtttttattgtttttgagacagggtctcacactgtgttgccaaggctggagtgcagtggcacaatcatggctcattatagcctcaaccgccagggctcagataatcctccctcctcagcctcctgagtagctaagactatgggtacggcaccatgcctggctaatttttaaatttttttggtagagatggggtcttgctcttttgtccagactggtcttgaactcctggcttcaggcaatcctccggcgtagccaggaccacaggtgcatgctaccatgctcagtttttttttttt

SEQ ID NO: 10973 - RNA, 3132 nt, Homo sapiens
  source 1..3132: mol_type = other RNA
ctgaatagctgggactacaggtgcacaccaccacacccagcaaatttttgtatttttaatagagacggcatttcaccatgttggtctcgaactcctgacctcatgatctgcctgctttggcctcccaaagtgctgggattacaggcgtgagccactgcactcagccacatgtggatttctttatgcgtggagtgcttctgccttgaaggcagtcagagccttccttagacccaggtgtcgtagtaactgtcatgcaggcctaggaaccccaactgccccggtgttccccagtgtggcccgcttggctcccccagccctcctgccgccctcatcctttcttctgtggtggctggaggcccccggggtctgatggagctgctcttggccacctgcaggttctcttctgctttgagcagtttgatgagctcaccctgctgcaccttcgtgagtttgacaagaagaagctgatctctgtggagacggacatagtcgtggatcactacaaggaggagaagtttgaggacaggtccccaggtcggcatcccctgctctctaggcgtggggctggtttccactccccgcacgcctctcctgccccgcagcgagggcttcctttgggttttcgtcagttgacctgggctcagccacccccgagaagagccttgtgggagcaccctggtgactggaggaaggtgcctcctggtttagatatcaggggtctgtccagtgctcctgccacggtggcttctggagctggcccagcttcttgagaggctgtgtatttttttaaagccctaaccaagttgtatgggcctcaggcaacctgaagcatcctttgaggttttacttttagatgaaaagcatcttgctagcttgtgtctccatcctggtgggagaggaggtgggagctggaagcatgctgcgtggcccccatggaagccggggagttgggatgcaggcctgagctccctgtcgcctgctcttccgcagccgccgagtgcctatcagagaaggagacggaggagctcatggcctggatgagaaatgtgctggggtcgcgtgtcaccaacgtgaaggtgaggctttcccggggatggaccaccacttggccgcagtgtccctaacaggctggccagctggtggctcccagtacctggcccgttgggtgtccttccagcagcagcagaagcccttggtgtcaggtggagaccctgtgggtccctgctcggcacgtgttgctcgggagtgccgctgaggcaggaaggccgtgtctttctcccagccctgctccagagcaggtgtgaactgagaacagttggtcactcaggccataggcagcctggaagttaaagggaagagccgagtcgggaacaacggcgcctcggagcagcatccctgcaaccacgatcctgtcataggcacagtgcgtgggtgtagctgtggtgtcagcgctgtcggggatcagccactggaaggtggggcttgtccacaggcggatggatgaccactgggagggtctcacatagctgcagcccgcattgaagtcgcccatcaacatgacgtcctccaagccccatttctcttggacatccaggtagacgtcatagagagcgtcgatctcggctactgcgtcccccggggccgcatgcaggggaacaatggcaaactccctgacctctgtgaaccgggagaagaacctgacaatggctggctctcggttgaaggtgtcgttcccgcagggctcgcagccatcatcgtagtagtagctgtccaccgcagacacctggtcaggcctgtacacgaacaggtagcgctccttatagctgttccgtcccagtggctcactgaccacgtagtgataggtgtctggtgcatcctgattgaggttgtccagcagcttccccacggcagtcaggtggctgtctctgacctcctggaccagggcgatgtcatagcggctcaggatctgcacaatgtagctgacgagggtggcattggacatcttggtctccccaaatgtctggatgttgaaggctgcgatcttcagggacacggccccctgcagtagggccgccagtgccagcagcgcccccagcagcttcatgcccctcatcctgagatgatggtgatgtcctcagagatgacgagaatgctgtcaagaatctggaatatcctttgatgacaattttctccttttgctccccaagcttccctgtgttgtgctgctgggcggctctccaggccttcaagctggggccttctgaacggtggccggctcctcgggtcctgggcaggagtgcttccccgtgagctcttccacaccagacgcagagcctgcggaaccttgccaaggcggcttcctaagctcctcccctgtggcccacatggaggggtggctgctggtcagggccacgccccccacagcgtggagctgcagcagggccatgctggccaccactagccaccctgccacagctgcagctgtggatggggcctcacgcaggagcagcaacagcacctgggggctggggatgagtctagcttggtgctgatccacccaaatccagagtgaccacatccgagtggccctgttgggcctgctccccactgtccaaagtccactggagtcacggtggagccatcgagacaggacagtggctctgcccttgagagctcatgggtgacgggctcctgtcctcgcttgagcccatgaggaggtgctgatcttcggaggtgcctgggcccaggagtgacagccacaggaagctagtgacatgcaacttgctggggaggccactacccaggctggcgctgtaccactcagcaagcttttgccatcttgctgttcccattcatattgtggtcactgagaggaagcttctcgggcccccaggccagatttggtgcctctcccggtccccctcacaccgtccactctccgctccacaggcaggtatgcccagagggggccgccgttgtatccgcgaacatttcctgagccagctggggaggaaccagactttatctcacagctgccacagtgccttaaactcgccctaactctttctcaaaaactaacagactccacctgaagcaagcgccgcttccgcctcgccccgcctcctgccgacc

SEQ ID NO: 10974 - RNA, 6875 nt, Homo sapiens
  source 1..6875: mol_type = other RNA
ctgaatagctgggactacaggtgcacaccaccacacccagcaaatttttgtatttttaatagagacggcatttcaccatgttggtctcgaactcctgacctcatgatctgcctgctttggcctcccaaagtgctgggattacaggcgtgagccactgcactcagccacatgtggatttctttatgcgtggagtgcttctgccttgaaggcagtcagagccttccttagacccaggtgtcgtagtaactgtcatgcaggcctaggaaccccaactgccccggtgttccccagtgtggcccgcttggctcccccagccctcctgccgccctcatcctttcttctgtggtggctggaggcccccggggtctgatggagctgctcttggccacctgcaggttctcttctgctttgagcagtttgatgagctcaccctgctgcaccttcgtgagtttgacaagaagaagctgatctctgtggagacggacatagtcgtggatcactacaaggaggagaagtttgaggacaggtccccaggtcggcatcccctgctctctaggcgtggggctggtttccactccccgcacgcctctcctgccccgcagcgagggcttcctttgggttttcgtcagttgacctgggctcagccacccccgagaagagccttgtgggagcaccctggtgactggaggaaggtgcctcctggtttagatatcaggggtctgtccagtgctcctgccacggtggcttctggagctggcccagcttcttgagaggctgtgtatttttttaaagccctaaccaagttgtatgggcctcaggcaacctgaagcatcctttgaggttttacttttagatgaaaagcatcttgctagcttgtgtctccatcctggtgggagaggaggtgggagctggaagcatgctgcgtggcccccatggaagccggggagttgggatgcaggcctgagctccctgtcgcctgctcttccgcagccgccgagtgcctatcagagaaggagacggaggagctcatggcctggatgagaaatgtgctggggtcgcgtgtcaccaacgtgaaggtgaggctttcccggggatggaccaccacttggccgcagtgtccctaacaggctggccagctggtggctcccagtacctggcccgttgggtgtccttccagcagcagcagaagcccttggtgtcaggtggagaccctgtgggtccctgctcggcacgtgttgctcgggagtgccgctgaggcaggaaggccgtgtctttctcccagccctgctccagagcaggtgtgaactgagaacagttggtcactcaggccataggcagcctggaagttaaagggaagagccgagtcgggaacaacggcgcctcggagcagcatccctgcaaccacgatcctgtcataggcacagtgcgtgggtgtagctgtggtgtcagcgctgtcggggatcagccactggaaggtggggcttgtccacaggcggatggatgaccactgggagggtctcacatagctgcagcccgcattgaagtcgcccatcaacatgacgtcctccaagccccatttctcttggacatccaggtagacgtcatagagagcgtcgatctcggctactgcgtcccccggggccgcatgcaggggaacaatggcaaactccctgacctctgtgaaccgggagaagaacctgacaatggctggctctcggttgaaggtgtcgttcccgcagggctcgcagccatcatcgtagtagtagctgtccaccgcagacacctggtcaggcctgtacacgaacaggtagcgctccttatagctgttccgtcccagtggctcactgaccacgtagtgataggtgtctggtgcatcctgattgaggttgtccagcagcttccccacggcagtcaggtggctgtctctgacctcctggaccagggcgatgtcatagcggctcaggatctgcacaatgtagctgacgagggtggcattggacatcttggtctccccaaatgtctggatgttgaaggctgcgatcttcagggacacggccccctgcagtagggccgccagtgccagcagcgcccccagcagcttcatgcccctcatcctgagatgatggtgatgtcctcagagatgacgagaatgctgtcaagaatctggaatatcctttgatgacaattttctccttttgctgcttaaagaaaaaaaagtagtctatgaagaaaggtctctgaagaagcacttcaaggccctggcagtgctgctgggctccggatcctgcacaggcagtgcgtgtctgggagttttaaaagttcaggcagctgtgaccttccctggggcaaatgtgagccgtcacctgagagtgcagaaaacaatggctctgtgtggctttccgcataggtgggttgctagcacgtgtttctttctgtaagcacaggtttcttgctgctgtaaaaactgcacctgataatcacgtttgcacttagttttaaaatgtctgataacaaggccaaaggttcctatcccgtgtcccttgcacgtgtggtggcccccatcttccaggatagggcagggatgggccaggtatgtgcgggagggtggggctgggctccagtctccctgtctcttgtctgggggccccaaggtcactttggacaaagaggccaaagccacatccaaagttgcaaatggagccccctggtggctgacagccatgactgctctgtggcccaggacacgcctgccttcctgattcatcgccatcaggtgcaggcaactctgcaggaggctggggagctcggaacaagcagtggtgggggcctgcagcaccagcgccgtggggccaggacaggtggggcctgcaaagcccaccccaattgccagccaagcagtggggagccttcttgaggtagacaataggctgtgtgtttaggcccaggggatcccgagtgaccaggtcacaagggcagggcagcagctaaaggccaggcctcaggtccagtaatttcttggttcttttgttttgggtttttattgtttttgagacagggtctcacactgtgttgccaaggctggagtgcagtggcacaatcatggctcattatagcctcaaccgccagggctcagataatcctccctcctcagcctcctgagtagctaagactatgggtacggcaccatgcctggctaatttttaaatttttttggtagagatggggtcttgctcttttgtccagactggtcttgaactcctggcttcaggcaatcctccggcgtagccaggaccacaggtgcatgctaccatgctcagtttttttttttttttttttttttttttttttttttgaggcggaatcttgctctgctgcccagcctggagtgcagtaatactatctcggctcactgcaacctctgcttcctgggttcaagcaattcttctgcctcagcctcccgagtagctgggattacaggcacgcaccaccacacccggctaatttttgtatttttagtagagacagggtttcaccatgttggtcacactggtctcaaactcgtgaccttgtgatccgcctgcctcggcctcccaaagtgctgggattacaggcgtgagccatcgcacccagcctattttttaagtttctcacagacacaaggtctccaagtcctgagcccaagcaatcttcccgcaaatgctgggattacaagtgtgagccaccgcaccccgccactcatttcttggaatctttgactttccattcgtattcatttcctgagactggtgaaactaccacaagtttggttgcttaaaataacagaaatggatcctctcaaaattccggagactggacgtctgaagtcagggagtcagtaggaccttgcgcctcctggaggctccgggcggttgggggatgctccttgccctccagtttctgcaggctgccagcaatccttggctttccttagttgtggctgcatcaccccagtctctgcctcttcttcttaagatctgtgcacctgcatttggggtcctcccagagagcagggaggatgtccttatctcaacagcctttactcacatctgcaagtccttttttgctacaaaaatcaacattcagaggttccagggctagggcacagctatcttttgagccacccctgggtcttgcccacttggaaggggctgtgctggccctccaaggacagccctgcacgtagcatctgtggtccccctgggggaggagggcctggaaggcttggcagaagtccaggcgggattcaggtatgagaactgcaggaaatgaatacaaatggggtctgcaggaggcctcaacggcaagagtcagcaggggccaaggtcgaaagtcaggaaagtgctcggtctggccagctggccatgaagcagaaggcaggcccagtggggactagaaacaggaaggtaaaccaccctccacaagactggcaccccattccataaagacacgccaacagacgcctctggctggcagcactggtgcactcatctgtccctcctattgagacggcgtctaccagatggaaacaccaccactcctcaggctgccagaggccccattgcaggcttttccaaaggtttcagcaatggttcttccctgtttttaatctctaagtctaggacagcctccagcacgtcaaaacccagcccccaagcaaggccaccggagtattcggtgtagggactagtcctctgcctttggtgtttgcctttcctggacacacatctgacagcgacccatcacggggaagggagtaaagctagagggcggccactgtcctccaccaagaaactgcctggtgcagcttccggcggggcacagggacaccaattatagctcacagagcaagtgcccaaccccctacgtgtgctcagcacgtgggacgagggttcccctctggtctgtcatcccctcctggctcttgaccaaatgctgccccatctgctttcaggaactcccaggcatagtgcccctgcttcctctacctgccagaaggaaggctggaacttgggcctcgcttgtacaaatggcgagtgctgcctgctgtgtggctgccctcaggacgggctttggtgagggcagcacagccctggaggagcctggtctgacatggggcccgtctgggatcactgttgggccttcaaccgtctggagcctctatgtcttcctctgatagattcccagaacaatcatttcaccttctaagaagccatcctgcccctgcagcctgtggcttgtggagtctccagcactctcacttctccctcgtggatctcttttctgtctgtgtcagtcaatgctgccatgtaacagccacctgcaaactcagtgtatacacatgcatttctctcacactgccaggtctgctggggtggctctgctgcctgggcctcgtcctggggctgggctggagagactgcagctccctgggcaccctcttcccacagtgtggaaggtggaggctcccagggcacaagcagaacacgtgccgccctaaggccaaggcggagctggctgctgtcgcttctgcccacattccatgggtgctgtcgagctgtaggtccaagccccacatcaggggagtgagtggggtacaatcctcccatgctgggccccactctggagataggcctggggaatgcccaagaaggaagcccagcccttctgggattttcacatccacagagaatgggtgctggcagccaacggcaacgaggagaaaagctgaccgccttctcagatcaggatgaggtgtttttacaccaaccccgaggatctgcagccttctcaggttaaattaaaccttgctttatagggtatcttccctctctctgccaggctgggttgtggcagtcactgaacaagcaattactgtgaaggtcgacgtggaaaaatgaggcaatgagggtggcggtgttctaccagattccaagttgaagaggtgctcgacaggcacacacatcccatgactaaacaaataacatgaacatttctctttatgtattacttttctagacatccactataagttgccaggacacaaatgcttattattggggtttacttatttaataaatggaactgtgggggatttctttttcttttctttttttttttttttttgaatgaccatataatctggacttactaactttaggtaacagtaagttaaaagatagaataaggtttcatattacaggaattcaaaaattgaccatataataaatgatgaagaaaactaacaataaacaggacaatgttcaaatagctcattggggccaaaagatcagcgtatatcctgcatcatctttcatgcaatgtctcagctttttttccctcaaacataaaggcagattaatacaaattagccttatttagaatattcatttacgtttccttctgaaattgatacttgagtggaagatgtattaataactcgtggtttctactgaaatttaagattccaccagatgatgctcagatttagacgatgctagagtaagacactactgggtgatgatttcaaagtatgagctgcaggtaaaatctaaaaggacatacataataacaaatgttttctaatttaaaagacatatagtaaatatccatgaattaactcacacaacctacttacaaacaaaactagaataaacaaaacttgtaggaaccaactccagttgatttcgccacttagcgggagcaagttctcaggcgggtcattttatttaaggatgacttgaaattttacaagaccaccttagctcccacatacgaaaactctttaagaattttttttttatcaactagaagttggggaaaacacaccgagaaataaa

SEQ ID NO: 10975 - RNA, 3737 nt, Homo sapiens
  source 1..3737: mol_type = other RNA
ctgaatagctgggactacaggtgcacaccaccacacccagcaaatttttgtatttttaatagagacggcatttcaccatgttggtctcgaactcctgacctcatgatctgcctgctttggcctcccaaagtgctgggattacaggcgtgagccactgcactcagccacatgtggatttctttatgcgtggagtgcttctgccttgaaggcagtcagagccttccttagacccaggtgtcgtagtaactgtcatgcaggcctaggaaccccaactgccccggtgttccccagtgtggcccgcttggctcccccagccctcctgccgccctcatcctttcttctgtggtggctggaggcccccggggtctgatggagctgctcttggccacctgcaggttctcttctgctttgagcagtttgatgagctcaccctgctgcaccttcgtgagtttgacaagaagaagctgatctctgtggagacggacatagtcgtggatcactacaaggaggagaagtttgaggacaggtccccaggtcggcatcccctgctctctaggcgtggggctggtttccactccccgcacgcctctcctgccccgcagcgagggcttcctttgggttttcgtcagttgacctgggctcagccacccccgagaagagccttgtgggagcaccctggtgactggaggaaggtgcctcctggtttagatatcaggggtctgtccagtgctcctgccacggtggcttctggagctggcccagcttcttgagaggctgtgtatttttttaaagccctaaccaagttgtatgggcctcaggcaacctgaagcatcctttgaggttttacttttagatgaaaagcatcttgctagcttgtgtctccatcctggtgggagaggaggtgggagctggaagcatgctgcgtggcccccatggaagccggggagttgggatgcaggcctgagctccctgtcgcctgctcttccgcagccgccgagtgcctatcagagaaggagacggaggagctcatggcctggatgagaaatgtgctggggtcgcgtgtcaccaacgtgaaggtgaggctttcccggggatggaccaccacttggccgcagtgtccctaacaggctggccagctggtggctcccagtacctggcccgttgggtgtccttccagcagcagcagaagcccttggtgtcaggtggagaccctgtgggtccctgctcggcacgtgttgctcgggagtgccgctgaggcaggaaggccgtgtctttctcccagccctgctccagagcaggtgtgaactgagaacagttggtcactcaggccataggcagcctggaagttaaagggaagagccgagtcgggaacaacggcgcctcggagcagcatccctgcaaccacgatcctgtcataggcacagtgcgtgggtgtagctgtggtgtcagcgctgtcggggatcagccactggaaggtggggcttgtccacaggcggatggatgaccactgggagggtctcacatagctgcagcccgcattgaagtcgcccatcaacatgacgtcctccaagccccatttctcttggacatccaggtagacgtcatagagagcgtcgatctcggctactgcgtcccccggggccgcatgcaggggaacaatggcaaactccctgacctctgtgaaccgggagaagaacctgacaatggctggctctcggttgaaggtgtcgttcccgcagggctcgcagccatcatcgtagtagtagctgtccaccgcagacacctggtcaggcctgtacacgaacaggtagcgctccttatagctgttccgtcccagtggctcactgaccacgtagtgataggtgtctggtgcatcctgattgaggttgtccagcagcttccccacggcagtcaggtggctgtctctgacctcctggaccagggcgatgtcatagcggctcaggatctgcacaatgtagctgacgagggtggcattggacatcttggtctccccaaatgtctggatgttgaaggctgcgatcttcagggacacggccccctgcagtagggccgccagtgccagcagcgcccccagcagcttcatgcccctcatcctgagatgatggtgatgtcctcagagatgacgagaatgctgtcaagaatctggaatatcctttgatgacaattttctccttttgcttctaagaagccatcctgcccctgcagcctgtggcttgtggagtctccagcactctcacttctccctcgtggatctcttttctgtctgtgtcagtcaatgctgccatgtaacagccacctgcaaactcagtgtatacacatgcatttctctcacactgccaggtctgctggggtggctctgctgcctgggcctcgtcctggggctgggctggagagactgcagctccctgggcaccctcttcccacagtgtggaaggtggaggctcccagggcacaagcagaacacgtgccgccctaaggccaaggcggagctggctgctgtcgcttctgcccacattccatgggtgctgtcgagctgtaggtccaagccccacatcaggggagtgagtggggtacaatcctcccatgctgggccccactctggagataggcctggggaatgcccaagaaggaagcccagcccttctgggattttcacatccacagagaatgggtgctggcagccaacggcaacgaggagaaaagctgaccgccttctcagatcaggatgaggtgtttttacaccaaccccgaggatctgcagccttctcaggttaaattaaacctccccaagcttccctgtgttgtgctgctgggcggctctccaggccttcaagctggggccttctgaacggtggccggctcctcgggtcctgggcaggagtgcttccccgtgagctcttccacaccagacgcagagcctgcggaaccttgccaaggcggcttcctaagctcctcccctgtggcccacatggaggggtggctgctggtcagggccacgccccccacagcgtggagctgcagcagggccatgctggccaccactagccaccctgccacagctgcagctgtggatggggcctcacgcaggagcagcaacagcacctgggggctggggatgagtctagcttggtgctgatccacccaaatccagagtgaccacatccgagtggccctgttgggcctgctccccactgtccaaagtccactggagtcacggtggagccatcgagacaggacagtggctctgcccttgagagctcatgggtgacgggctcctgtcctcgcttgagcccatgaggaggtgctgatcttcggaggtgcctgggcccaggagtgacagccacaggaagctagtgacatgcaacttgctggggaggccactacccaggctggcgctgtaccactcagcaagcttttgccatcttgctgttcccattcatattgtggtcactgagaggaagcttctcgggcccccaggccagatttggtgcctctcccggtccccctcacaccgtccactctccgctccacaggcaggtatgcccagagggggccgccgttgtatccgcgaacatttcctgagccagctggggaggaaccagactttatctcacagctgccacagtgccttaaactcgccctaactctttctcaaaaactaacagactccacctgaagcaagcgccgcttccgcctcgccccgcctcctgccgacc

SEQ ID NO: 10976 - RNA, 2934 nt, Homo sapiens
  source 1..2934: mol_type = other RNA
ctgaatagctgggactacaggtgcacaccaccacacccagcaaatttttgtatttttaatagagacggcatttcaccatgttggtctcgaactcctgacctcatgatctgcctgctttggcctcccaaagtgctgggattacaggcgtgagccactgcactcagccacatgtggatttctttatgcgtggagtgcttctgccttgaaggcagtcagagccttccttagacccaggtgtcgtagtaactgtcatgcaggcctaggaaccccaactgccccggtgttccccagtgtggcccgcttggctcccccagccctcctgccgccctcatcctttcttctgtggtggctggaggcccccggggtctgatggagctgctcttggccacctgcaggttctcttctgctttgagcagtttgatgagctcaccctgctgcaccttcgtgagtttgacaagaagaagctgatctctgtggagacggacatagtcgtggatcactacaaggaggagaagtttgaggacaggtccccaggtcggcatcccctgctctctaggcgtggggctggtttccactccccgcacgcctctcctgccccgcagcgagggcttcctttgggttttcgtcagttgacctgggctcagccacccccgagaagagccttgtgggagcaccctggtgactggaggaaggtgcctcctggtttagatatcaggggtctgtccagtgctcctgccacggtggcttctggagctggcccagcttcttgagaggctgtgtatttttttaaagccctaaccaagttgtatgggcctcaggcaacctgaagcatcctttgaggttttacttttagatgaaaagcatcttgctagcttgtgtctccatcctggtgggagaggaggtgggagctggaagcatgctgcgtggcccccatggaagccggggagttgggatgcaggcctgagctccctgtcgcctgctcttccgcagccgccgagtgcctatcagagaaggagacggaggagctcatggcctggatgagaaatgtgctggggtcgcgtgtcaccaacgtgaaggtgaggctttcccggggatggaccaccacttggccgcagtgtccctaacaggctggccagctggtggctcccagtacctggcccgttgggtgtccttccagcagcagcagaagcccttggtgtcaggtggagaccctgtgggtccctgctcggcacgtgttgctcgggagtgccgctgaggcaggaaggccgtgtctttctcccagccctgctccagagcaggtgtgaactgagaacagttggtcactcaggccataggcagcctggaagttaaagggaagagccgagtcgggaacaacggcgcctcggagcagcatccctgcaaccacgatcctgtcataggcacagtgcgtgggtgtagctgtggtgtcagcgctgtcggggatcagccactggaaggtggggcttgtccacaggcggatggatgaccactgggagggtctcacatagctgcagcccgcattgaagtcgcccatcaacatgacgtcctgtgaaccgggagaagaacctgacaatggctggctctcggttgaaggtgtcgttcccgcagggctcgcagccatcatcgtagtagtagctgtccaccgcagacacctggtcaggcctgtacacgaacaggtagcgctccttatagctgttccgtcccagtggctcactgaccacgtagtgataggtgtctggtgcatccctgcacaatgtagctgacgagggtggcattggacatcttggtctccccaaatgtctggatgttgaaggctgcgatcttcagggacacggccccctgcagtagggccgccagtgccagcagcgcccccagcagcttcatgcccctcatcctgagatgatggtgatgtcctcagagatgacgagaatgctgtcaagaatctggaatatcctttgatgacaattttctccttttgctccccaagcttccctgtgttgtgctgctgggcggctctccaggccttcaagctggggccttctgaacggtggccggctcctcgggtcctgggcaggagtgcttccccgtgagctcttccacaccagacgcagagcctgcggaaccttgccaaggcggcttcctaagctcctcccctgtggcccacatggaggggtggctgctggtcagggccacgccccccacagcgtggagctgcagcagggccatgctggccaccactagccaccctgccacagctgcagctgtggatggggcctcacgcaggagcagcaacagcacctgggggctggggatgagtctagcttggtgctgatccacccaaatccagagtgaccacatccgagtggccctgttgggcctgctccccactgtccaaagtccactggagtcacggtggagccatcgagacaggacagtggctctgcccttgagagctcatgggtgacgggctcctgtcctcgcttgagcccatgaggaggtgctgatcttcggaggtgcctgggcccaggagtgacagccacaggaagctagtgacatgcaacttgctggggaggccactacccaggctggcgctgtaccactcagcaagcttttgccatcttgctgttcccattcatattgtggtcactgagaggaagcttctcgggcccccaggccagatttggtgcctctcccggtccccctcacaccgtccactctccgctccacaggcaggtatgcccagagggggccgccgttgtatccgcgaacatttcctgagccagctggggaggaaccagactttatctcacagctgccacagtgccttaaactcgccctaactctttctcaaaaactaacagactccacctgaagcaagcgccgcttccgcctcgccccgcctcctgccgaccggaa

SEQ ID NO: 10977 - RNA, 2962 nt, Homo sapiens
  source 1..2962: mol_type = other RNA
ctgaatagctgggactacaggtgcacaccaccacacccagcaaatttttgtatttttaatagagacggcatttcaccatgttggtctcgaactcctgacctcatgatctgcctgctttggcctcccaaagtgctgggattacaggcgtgagccactgcactcagccacatgtggatttctttatgcgtggagtgcttctgccttgaaggcagtcagagccttccttagacccaggtgtcgtagtaactgtcatgcaggcctaggaaccccaactgccccggtgttccccagtgtggcccgcttggctcccccagccctcctgccgccctcatcctttcttctgtggtggctggaggcccccggggtctgatggagctgctcttggccacctgcaggttctcttctgctttgagcagtttgatgagctcaccctgctgcaccttcgtgagtttgacaagaagaagctgatctctgtggagacggacatagtcgtggatcactacaaggaggagaagtttgaggacaggtccccaggtcggcatcccctgctctctaggcgtggggctggtttccactccccgcacgcctctcctgccccgcagcgagggcttcctttgggttttcgtcagttgacctgggctcagccacccccgagaagagccttgtgggagcaccctggtgactggaggaaggtgcctcctggtttagatatcaggggtctgtccagtgctcctgccacggtggcttctggagctggcccagcttcttgagaggctgtgtatttttttaaagccctaaccaagttgtatgggcctcaggcaacctgaagcatcctttgaggttttacttttagatgaaaagcatcttgctagcttgtgtctccatcctggtgggagaggaggtgggagctggaagcatgctgcgtggcccccatggaagccggggagttgggatgcaggcctgagctccctgtcgcctgctcttccgcagccgccgagtgcctatcagagaaggagacggaggagctcatggcctggatgagaaatgtgctggggtcgcgtgtcaccaacgtgaaggtgaggctttcccggggatggaccaccacttggccgcagtgtccctaacaggctggccagctggtggctcccagtacctggcccgttgggtgtccttccagcagcagcagaagcccttggtgtcaggtggagaccctgtgggtccctgctcggcacgtgttgctcgggagtgccgctgaggcaggaaggccgtgtctttctcccagccctgctccagagcaggtgtgaactgagaacagttggtcactcaggccataggcagcctggaagttaaagggaagagccgagtcgggaacaacggcgcctcggagcagcatccctgcaaccacgatcctgtcataggcacagtgcgtgggtgtagctgtggtgtcagcgctgtcggggatcagccactggaaggtggggcttgtccacaggcggatggatgaccactgggagggtctcacatagctgcagcccgcattgaagtcgcccatcaacatgacgtcctgtgaaccgggagaagaacctgacaatggctggctctcggttgaaggtgtcgttcccgcagggctcgcagccatcatcgtagtagtagctgtccaccgcagacacctggtcaggcctgtacacgaacaggtagcgctccttatagctgttccgtcccagtggctcactgaccacgtagtgataggtgtctggtgcatccctgcacaatgtagctgacgagggtggcattggacatcttggtctccccaaatgtctggatgttgaaggctgcgatcttcagggacacggccccctgcagtagggccgccagtgccagcagcgcccccagcagcttcatgcccctcatcctgagatgatggtgatgtcctcagagatgacgagaatgctgtcaagaatctggaatatcctttgatgacaattttctccttttgctgagagtgcagaaaacaatggctctgtgtggctttccgcataggtgggttgctagcacgtgtttctttctgtaagcacaggtttcttgctgctgtaaaaactgcacctgataatcacgtttgcacttagttttaaaatgtctgataacaaggccaaaggttcctatcccgtgtcccttgcacgtgtggtggcccccatcttccaggatagggcagggatgggccaggtatgtgcgggagggtggggctgggctccagtctccctgtctcttgtctgggggccccaaggtcactttggacaaagaggccaaagccacatccaaagttgcaaatggagccccctggtggctgacagccatgactgctctgtggcccaggacacgcctgccttcctgattcatcgccatcaggtgcaggcaactctgcaggaggctggggagctcggaacaagcagtggtgggggcctgcagcaccagcgccgtggggccaggacaggtggggcctgcaaagcccaccccaattgccagccaagcagtggggagccttcttgaggtagacaataggctgtgtgtttaggcccaggggatcccgagtgaccaggtcacaagggcagggcagcagctaaaggccaggcctcaggtccagtaatttcttggttcttttgttttgggtttttattgtttttgagacagggtctcacactgtgttgccaaggctggagtgcagtggcacaatcatggctcattatagcctcaaccgccagggctcagataatcctccctcctcagcctcctgagtagctaagactatgggtacggcaccatgcctggctaatttttaaatttttttggtagagatggggtcttgctcttttgtccagactggtcttgaactcctggcttcaggcaatcctccggcgtagccaggaccacaggtgcatgctaccatgctcagtttttttttttt

SEQ ID NO: 10978 - RNA, 3539 nt, Homo sapiens
  source 1..3539: mol_type = other RNA
ctgaatagctgggactacaggtgcacaccaccacacccagcaaatttttgtatttttaatagagacggcatttcaccatgttggtctcgaactcctgacctcatgatctgcctgctttggcctcccaaagtgctgggattacaggcgtgagccactgcactcagccacatgtggatttctttatgcgtggagtgcttctgccttgaaggcagtcagagccttccttagacccaggtgtcgtagtaactgtcatgcaggcctaggaaccccaactgccccggtgttccccagtgtggcccgcttggctcccccagccctcctgccgccctcatcctttcttctgtggtggctggaggcccccggggtctgatggagctgctcttggccacctgcaggttctcttctgctttgagcagtttgatgagctcaccctgctgcaccttcgtgagtttgacaagaagaagctgatctctgtggagacggacatagtcgtggatcactacaaggaggagaagtttgaggacaggtccccaggtcggcatcccctgctctctaggcgtggggctggtttccactccccgcacgcctctcctgccccgcagcgagggcttcctttgggttttcgtcagttgacctgggctcagccacccccgagaagagccttgtgggagcaccctggtgactggaggaaggtgcctcctggtttagatatcaggggtctgtccagtgctcctgccacggtggcttctggagctggcccagcttcttgagaggctgtgtatttttttaaagccctaaccaagttgtatgggcctcaggcaacctgaagcatcctttgaggttttacttttagatgaaaagcatcttgctagcttgtgtctccatcctggtgggagaggaggtgggagctggaagcatgctgcgtggcccccatggaagccggggagttgggatgcaggcctgagctccctgtcgcctgctcttccgcagccgccgagtgcctatcagagaaggagacggaggagctcatggcctggatgagaaatgtgctggggtcgcgtgtcaccaacgtgaaggtgaggctttcccggggatggaccaccacttggccgcagtgtccctaacaggctggccagctggtggctcccagtacctggcccgttgggtgtccttccagcagcagcagaagcccttggtgtcaggtggagaccctgtgggtccctgctcggcacgtgttgctcgggagtgccgctgaggcaggaaggccgtgtctttctcccagccctgctccagagcaggtgtgaactgagaacagttggtcactcaggccataggcagcctggaagttaaagggaagagccgagtcgggaacaacggcgcctcggagcagcatccctgcaaccacgatcctgtcataggcacagtgcgtgggtgtagctgtggtgtcagcgctgtcggggatcagccactggaaggtggggcttgtccacaggcggatggatgaccactgggagggtctcacatagctgcagcccgcattgaagtcgcccatcaacatgacgtcctgtgaaccgggagaagaacctgacaatggctggctctcggttgaaggtgtcgttcccgcagggctcgcagccatcatcgtagtagtagctgtccaccgcagacacctggtcaggcctgtacacgaacaggtagcgctccttatagctgttccgtcccagtggctcactgaccacgtagtgataggtgtctggtgcatccctgcacaatgtagctgacgagggtggcattggacatcttggtctccccaaatgtctggatgttgaaggctgcgatcttcagggacacggccccctgcagtagggccgccagtgccagcagcgcccccagcagcttcatgcccctcatcctgagatgatggtgatgtcctcagagatgacgagaatgctgtcaagaatctggaatatcctttgatgacaattttctccttttgcttctaagaagccatcctgcccctgcagcctgtggcttgtggagtctccagcactctcacttctccctcgtggatctcttttctgtctgtgtcagtcaatgctgccatgtaacagccacctgcaaactcagtgtatacacatgcatttctctcacactgccaggtctgctggggtggctctgctgcctgggcctcgtcctggggctgggctggagagactgcagctccctgggcaccctcttcccacagtgtggaaggtggaggctcccagggcacaagcagaacacgtgccgccctaaggccaaggcggagctggctgctgtcgcttctgcccacattccatgggtgctgtcgagctgtaggtccaagccccacatcaggggagtgagtggggtacaatcctcccatgctgggccccactctggagataggcctggggaatgcccaagaaggaagcccagcccttctgggattttcacatccacagagaatgggtgctggcagccaacggcaacgaggagaaaagctgaccgccttctcagatcaggatgaggtgtttttacaccaaccccgaggatctgcagccttctcaggttaaattaaacctccccaagcttccctgtgttgtgctgctgggcggctctccaggccttcaagctggggccttctgaacggtggccggctcctcgggtcctgggcaggagtgcttccccgtgagctcttccacaccagacgcagagcctgcggaaccttgccaaggcggcttcctaagctcctcccctgtggcccacatggaggggtggctgctggtcagggccacgccccccacagcgtggagctgcagcagggccatgctggccaccactagccaccctgccacagctgcagctgtggatggggcctcacgcaggagcagcaacagcacctgggggctggggatgagtctagcttggtgctgatccacccaaatccagagtgaccacatccgagtggccctgttgggcctgctccccactgtccaaagtccactggagtcacggtggagccatcgagacaggacagtggctctgcccttgagagctcatgggtgacgggctcctgtcctcgcttgagcccatgaggaggtgctgatcttcggaggtgcctgggcccaggagtgacagccacaggaagctagtgacatgcaacttgctggggaggccactacccaggctggcgctgtaccactcagcaagcttttgccatcttgctgttcccattcatattgtggtcactgagaggaagcttctcgggcccccaggccagatttggtgcctctcccggtccccctcacaccgtccactctccgctccacaggcaggtatgcccagagggggccgccgttgtatccgcgaacatttcctgagccagctggggaggaaccagactttatctcacagctgccacagtgccttaaactcgccctaactctttctcaaaaactaacagactccacctgaagcaagcgccgcttccgcctcgccccgcctcctgccgaccggaa

SEQ ID NO: 10979 - RNA, 1855 nt, Homo sapiens
  source 1..1855: mol_type = other RNA
ctgaatagctgggactacaggtgcacaccaccacacccagcaaatttttgtatttttaatagagacggcatttcaccatgttggtctcgaactcctgacctcatgatctgcctgctttggcctcccaaagtgctgggattacaggcgtgagccactgcactcagccacatgtggatttctttatgcgtggagtgcttctgccttgaaggcagtcagagccttccttagacccaggtgtcgtagtaactgtcatgcaggcctaggaaccccaactgccccggtgttccccagtgtggcccgcttggctcccccagccctcctgccgccctcatcctttcttctgtggtggctggaggcccccggggtctgatggagctgctcttggccacctgcaggttctcttctgctttgagcagtttgatgagctcaccctgctgcaccttcgtgagtttgacaagaagaagctgatctctgtggagacggacatagtcgtggatcactacaaggaggagaagtttgaggacaggtccccaggtcggcatcccctgctctctaggcgtggggctggtttccactccccgcacgcctctcctgccccgcagcgagggcttcctttgggttttcgtcagttgacctgggctcagccacccccgagaagagccttgtgggagcaccctggtgactggaggaaggtgcctcctggtttagatatcaggggtctgtccagtgctcctgccacggtggcttctggagctggcccagcttcttgagaggctgtgtatttttttaaagccctaaccaagttgtatgggcctcaggcaacctgaagcatcctttgaggttttacttttagatgaaaagcatcttgctagcttgtgtctccatcctggtgggagaggaggtgggagctggaagcatgctgcgtggcccccatggaagccggggagttgggatgcaggcctgagctccctgtcgcctgctcttccgcagccgccgagtgcctatcagagaaggagacggaggagctcatggcctggatgagaaatgtgctggggtcgcgtgtcaccaacgtgaaggtgaggctttcccggggatggaccaccacttggccgcagtgtccctaacaggctggccagctggtggctcccagtacctggcccgttgggtgtccttccagcagcagcagaagcccttggtgtcaggtggagaccctgtgggtccctgctcggcacgtgttgctcgggagtgccgctgaggcaggaaggccgtgtctttctcccagccctgctccagagcaggtgtgaactgagaacagttggtcactcaggccataggcagcctggaagttaaagggaagagccgagtcgggaacaacggcgcctcggagcagcatccctgcaaccacgatcctgtcataggcacagtgcgtgggtgtagctgtggtgtcagcgctgtcggggatcagccactggaaggtggggcttgtccacaggcggatggatgaccactgggagggtctcacatagctgcagcccgcattgaagtcgcccatcaacatgacgtcctgtgaaccgggagaagaacctgacaatggctggctctcggttgaaggtgtcgttcccgcagggctcgcagccatcatcgtagtagtagctgtccaccgcagacacctggtcaggcctgtacacgaacaggtagcgctccttatagctgttccgtcccagtggctcactgaccacgtagtgataggtgtctggtgcatcccttcctatgaccctgccactgtcacccactgattgaggttgtccagcagcttccccacggcagtcaggtggctgtctctgacctcctggac

SEQ ID NO: 10980 - RNA, 3216 nt, Homo sapiens
  source 1..3216: mol_type = other RNA
ctgaatagctgggactacaggtgcacaccaccacacccagcaaatttttgtatttttaatagagacggcatttcaccatgttggtctcgaactcctgacctcatgatctgcctgctttggcctcccaaagtgctgggattacaggcgtgagccactgcactcagccacatgtggatttctttatgcgtggagtgcttctgccttgaaggcagtcagagccttccttagacccaggtgtcgtagtaactgtcatgcaggcctaggaaccccaactgccccggtgttccccagtgtggcccgcttggctcccccagccctcctgccgccctcatcctttcttctgtggtggctggaggcccccggggtctgatggagctgctcttggccacctgcaggttctcttctgctttgagcagtttgatgagctcaccctgctgcaccttcgtgagtttgacaagaagaagctgatctctgtggagacggacatagtcgtggatcactacaaggaggagaagtttgaggacaggtccccaggtcggcatcccctgctctctaggcgtggggctggtttccactccccgcacgcctctcctgccccgcagcgagggcttcctttgggttttcgtcagttgacctgggctcagccacccccgagaagagccttgtgggagcaccctggtgactggaggaaggtgcctcctggtttagatatcaggggtctgtccagtgctcctgccacggtggcttctggagctggcccagcttcttgagaggctgtgtatttttttaaagccctaaccaagttgtatgggcctcaggcaacctgaagcatcctttgaggttttacttttagatgaaaagcatcttgctagcttgtgtctccatcctggtgggagaggaggtgggagctggaagcatgctgcgtggcccccatggaagccggggagttgggatgcaggcctgagctccctgtcgcctgctcttccgcagccgccgagtgcctatcagagaaggagacggaggagctcatggcctggatgagaaatgtgctggggtcgcgtgtcaccaacgtgaaggtgaggctttcccggggatggaccaccacttggccgcagtgtccctaacaggctggccagctggtggctcccagtacctggcccgttgggtgtccttccagcagcagcagaagcccttggtgtcaggtggagaccctgtgggtccctgctcggcacgtgttgctcgggagtgccgctgaggcaggaaggccgtgtctttctcccagccctgctccagagcaggtgtgaactgagaacagttggtcactcaggccataggcagcctggaagttaaagggaagagccgagtcgggaacaacggcgcctcggagcagcatccctgcaaccacgatcctgtcataggcacagtgcgtgggtgtagctgtggtgtcagcgctgtcggggatcagccactggaaggtggggcttgtccacaggcggatggatgaccactgggagggtctcacatagctgcagcccgcattgaagtcgcccatcaacatgacgtcctgtgaaccgggagaagaacctgacaatggctggctctcggttgaaggtgtcgttcccgcagggctcgcagccatcatcgtagtagtagctgtccaccgcagacacctggtcaggcctgtacacgaacaggtagcgctccttatagctgttccgtcccagtggctcactgaccacgtagtgataggtgtctggtgcatcctgattgaggttgtccagcagcttccccacggcagtcaggtggctgtctctgacctcctggaccagggcgatgtcatagcggctcaggatctgcacaatgtagctgacgagggtggcattggacatcttggtctccccaaatgtctggatgttgaaggctgcgatcttcagggacacggccccctgcagtagggccgccagtgccagcagcgcccccagcagcttcatgcccctcatcctgagatgatggtgatgtcctcagagatgacgagaatgctgtcaagaatctggaatatcctttgatgacaattttctccttttgctgcttaaagaaaaaaaagtagtctatgaagaaaggtctctgaagaagcacttcaaggccctggcagtgctgctgggctccggatcctgcacaggcagtgcgtgtctgggagttttaaaagttcaggcagctgtgaccttccctggggcaaatgtgagccgtcacctgagagtgcagaaaacaatggctctgtgtggctttccgcataggtgggttgctagcacgtgtttctttctgtaagcacaggtttcttgctgctgtaaaaactgcacctgataatcacgtttgcacttagttttaaaatgtctgataacaaggccaaaggttcctatcccgtgtcccttgcacgtgtggtggcccccatcttccaggatagggcagggatgggccaggtatgtgcgggagggtggggctgggctccagtctccctgtctcttgtctgggggccccaaggtcactttggacaaagaggccaaagccacatccaaagttgcaaatggagccccctggtggctgacagccatgactgctctgtggcccaggacacgcctgccttcctgattcatcgccatcaggtgcaggcaactctgcaggaggctggggagctcggaacaagcagtggtgggggcctgcagcaccagcgccgtggggccaggacaggtggggcctgcaaagcccaccccaattgccagccaagcagtggggagccttcttgaggtagacaataggctgtgtgtttaggcccaggggatcccgagtgaccaggtcacaagggcagggcagcagctaaaggccaggcctcaggtccagtaatttcttggttcttttgttttgggtttttattgtttttgagacagggtctcacactgtgttgccaaggctggagtgcagtggcacaatcatggctcattatagcctcaaccgccagggctcagataatcctccctcctcagcctcctgagtagctaagactatgggtacggcaccatgcctggctaatttttaaatttttttggtagagatggggtcttgctcttttgtccagactggtcttgaactcctggcttcaggcaatcctccggcgtagccaggaccacaggtgcatgctaccatgctcagtttttttttttt

SEQ ID NO: 10981 - RNA, 3164 nt, Homo sapiens
  source 1..3164: mol_type = other RNA
ctgaatagctgggactacaggtgcacaccaccacacccagcaaatttttgtatttttaatagagacggcatttcaccatgttggtctcgaactcctgacctcatgatctgcctgctttggcctcccaaagtgctgggattacaggcgtgagccactgcactcagccacatgtggatttctttatgcgtggagtgcttctgccttgaaggcagtcagagccttccttagacccaggtgtcgtagtaactgtcatgcaggcctaggaaccccaactgccccggtgttccccagtgtggcccgcttggctcccccagccctcctgccgccctcatcctttcttctgtggtggctggaggcccccggggtctgatggagctgctcttggccacctgcaggttctcttctgctttgagcagtttgatgagctcaccctgctgcaccttcgtgagtttgacaagaagaagctgatctctgtggagacggacatagtcgtggatcactacaaggaggagaagtttgaggacaggtccccaggtcggcatcccctgctctctaggcgtggggctggtttccactccccgcacgcctctcctgccccgcagcgagggcttcctttgggttttcgtcagttgacctgggctcagccacccccgagaagagccttgtgggagcaccctggtgactggaggaaggtgcctcctggtttagatatcaggggtctgtccagtgctcctgccacggtggcttctggagctggcccagcttcttgagaggctgtgtatttttttaaagccctaaccaagttgtatgggcctcaggcaacctgaagcatcctttgaggttttacttttagatgaaaagcatcttgctagcttgtgtctccatcctggtgggagaggaggtgggagctggaagcatgctgcgtggcccccatggaagccggggagttgggatgcaggcctgagctccctgtcgcctgctcttccgcagccgccgagtgcctatcagagaaggagacggaggagctcatggcctggatgagaaatgtgctggggtcgcgtgtcaccaacgtgaaggtgaggctttcccggggatggaccaccacttggccgcagtgtccctaacaggctggccagctggtggctcccagtacctggcccgttgggtgtccttccagcagcagcagaagcccttggtgtcaggtggagaccctgtgggtccctgctcggcacgtgttgctcgggagtgccgctgaggcaggaaggccgtgtctttctcccagccctgctccagagcaggtgtgaactgagaactgagctcctgtgtcccatcctcatgtggctgtgcaagggaggacacataccagttggtcactcaggccataggcagcctggaagttaaagggaagagccgagtcgggaacaacggcgcctcggagcagcatccctgcaaccacgatcctgtcataggcacagtgcgtgggtgtagctgtggtgtcagcgctgtcggggatcagccactggaaggtggggcttgtccacaggcggatggatgaccactgggagggtctcacatagctgcagcccgcattgaagtcgcccatcaacatgacgtcctccaagccccatttctcttggacatccaggtagacgtcatagagagcgtcgatctcggctactgcgtcccccggggccgcatgcaggggaacaatggcaaactccctgacctctgtgaaccgggagaagaacctgacaatggctggctctcggttgaaggtgtcgttcccgcagggctcgcagccatcatcgtagtagtagctgtccaccgcagacacctggtcaggcctgtacacgaacaggtagcgctccttatagctgttccgtcccagtggctcactgaccacgtagtgataggtgtctggtgcatcctgattgaggttgtccagcagcttccccacggcagtcaggtggctgtctctgacctcctggaccagggcgatgtcatagcggctcaggatctgcacaatgtagctgacgagggtggcattggacatcttggtctccccaaatgtctggatgttgaaggctgcgatcttcagggacacggccccctgcagtagggccgccagtgccagcagcgcccccagcagcttcatgcccctcatcctgagatgatggtgatgtcctcagagatgacgagaatgctgtcaagaatctggaatatcctttgatgacaattttctccttttgctccccaagcttccctgtgttgtgctgctgggcggctctccaggccttcaagctggggccttctgaacggtggccggctcctcgggtcctgggcaggagtgcttccccgtgagctcttccacaccagacgcagagcctgcggaaccttgccaaggcggcttcctaagctcctcccctgtggcccacatggaggggtggctgctggtcagggccacgccccccacagcgtggagctgcagcagggccatgctggccaccactagccaccctgccacagctgcagctgtggatggggcctcacgcaggagcagcaacagcacctgggggctggggatgagtctagcttggtgctgatccacccaaatccagagtgaccacatccgagtggccctgttgggcctgctccccactgtccaaagtccactggagtcacggtggagccatcgagacaggacagtggctctgcccttgagagctcatgggtgacgggctcctgtcctcgcttgagcccatgaggaggtgctgatcttcggaggtgcctgggcccaggagtgacagccacaggaagctagtgacatgcaacttgctggggaggccactacccaggctggcgctgtaccactcagcaagcttttgccatcttgctgttcccattcatattgtggtcactgagaggaagcttctcgggcccccaggccagatttggtgcctctcccggtccccctcacaccgtccactctccgctccacaggcaggtatgcccagagggggccgccgttgtatccgcgaacatttcctgagccagctggggaggaaccagactttatctcacagctgccacagtgccttaaactcgccctaactctttctcaaaaactaacagactccacctgaagcaagcgccgcttccgcctc

SEQ ID NO: 10982 - RNA, 10034 nt, Homo sapiens
  source 1..10034: mol_type = other RNA
ctgaatagctgggactacaggtgcacaccaccacacccagctaatttttttatttttgtagggactacaggtgcacaccaccacacccagctaatttttttatttttgtatttttacttttcaccatgtcggtcaggctggtctcaaactcctgacctcaggtgatctgcccacctcagcctcccaaagtgccgggattacaggcatgagccaccgtgcccagcccttaattgctgtctgaaccttttttttttttttcaacctgacctgaggcatcaattcaggcacagtataactctgaccagtaagcggaagctaacccaaatgctttccagggctgaggggacatcatgagagttgtggtcatgtacagaagcacagtcccaggggcacaggtggtacccctgtaaacaaagaatttgcaatattagggcacctcaagcaggacatccattaggctgtacaggtgaacagacctcctaccaggggaactcctgcccaagtgtttccagtcccatctgaaaagttcccagagtccttggcttccaagggactgcctgaaggcagtgagtcccaaacagttttgcttgttcaggatacaagttgatccatctcatgagcatggatgacatttgtgggagatcttcatggaaagcatagaagctagacccactctgttgtcagtctgaactcaaagcactcacagcacatggaaaggcagcactgggaattttccttcagcaagaggaggcttccagggatcaagcctccccaggtgccaggctttaattattttctccaatattacaaaaacagtcgtgccctgttcagcaatcataacattgcattttttcaaccatctcttactctcagctaggcctttcctctggaagggttgtatgtaagaggcacaaaagcatttttgtagataaacttttttttttttttttttgagatatggtctggctctgttgcccaggctagagtgcggtggcacgattttggctcactgcaacctccgcctcctgggctcaagccatcctcctacctcagcctcctaagtagctggaaccaaaggcacatgccatcatgtccagctaatttttgcattttttgtagacacaggatttcaccatgttgccaggctggtcttgaactcctgaactcaagcaatctgcccacctcggcctcccaaagtgctgggatcatatgcatccatcactgcgcctggccaacatttttttttttaactatcatcctagagttcaagtagataaacgtttttatgcaacttaaccagaaagacattcagaaattggtaattatgtgtggagggttgaattatgtccccacaaaaattcatgctgaagccctaaccatctacctgtacctcaaaatgtgagtatatttgaagataggccctgaagaggtaactaagttaaaatgggattgttaggatgggccctaatccaacctgagtggtatccttattaaaagagaagattaggacacagacacccagacagagggaccatacaaggacacagtaagaaggcagccatctgcaagccaagcagagaggcctcagaagaatctaaagctgtcgacaccttgtcctggactttcagcctccagaactgcaggaaaataagtttctattgtgtaagtcactcagtttgtggtactttgttatggtatccttagcaaactaataaaggatgaaaccctgaatttttaaaaatttcaaaatgtgtttacataatcttctaccccttttgtcctgattattcaatgagcagactagaaaagcctaatacctttctggggacagctacgttttaataatccacctaccttactaagctgtgtgtgctgggagaaaagtgagggaagtagagtcaggctgtcagtccactgttgcaagctgcaactaatcccaaaagctgaatgcaacaagtcaacagcagtgagagaagccccagagaaggtttgagtctggtctgtcaaaagcaggaggagaggtcatagtccttgcgatgtgcccttccccagcttggagcgtttggcaaatattagaagttaggaatgcaattagcctctgtattagagacaaagagcctatcagcagcttgatcttagatggtcccattagagaataagcccttttcagccaggttccaggacgttttcatagtttagcgctccacggagggggtccttaatctccaacggccccaacgtctgagtcctggtcattgagcctgtgcctgctttcagttcagcatagctcgtgttgaggctaaaacagctcaaggcagacagtagcaggtttcagcttagagtcagggccaggcaattaggatctgagaatttgagattctcaacaagcagctgcttttcttcagcagcagtgaaggcatgctgcatggccagacagctgtggtccaagtgacatgcaaggctgcctttttatcttgttggtcttagagtccaattgacccactcaaaaaaaatgcatattagactagacaatcatcagcctctaaggggagacatttgattttgacaagggttcattagcaatttaactgtattttcattttccaaacagattgcttctctttacatgttgtctccctctttcccgaggctccagtaagcacgaatcacagcaaaaataatcagttacagcctgttctggttccaatatccgaagaatttaaattccaacctatccactagtggcaaaaaactagaaagctgtatcccactaacacctttcatattttatttttgagtagctttatttgattagggtgatccctctagcatttatgaaattaacaagcataaaactttttttttaagagatgagtagctgggactacaggcgcacgccactgcgtccagctaaggtatgttttttaagcaatgaaatcaaccagtaaaaacaagttcaaatatttttcattcacacactcaaggcctgctgagcatccactgcatgtgttttacttgttccattagaaaggtttattaaaaaatggcggggcacagtggctcatgactgtaatcccagcacttagggaggccaagatcgcttgagcccaggagttcaagactagtctgggcaacatggtaaaaccctgtctctatttaaaaaataaacaaatacaagcaagtttttttttaaaaaatgatatattaaagaaaatcctcctaattctcttatgtcttttcatagctgtttccatgttctcatattcccatccttgtcaacatggaatttttgttgttgttgttgtggtttttttttttttttttgagacggagtctcgctctgtcgcccaggctggagtgcagtggcacaattacagctcactgcaagctccgccccctgggttcgcgccattctcctgcctcagcctcccaagtagctgggaatacaggcacccgccaccatgcctggctaatttttttgtatttttagtagagatggggtttcactgtgttagccaggatggtcttgatctcctgacctcgtgatctgcccacctcggcctcccgaagtgatgggattacaggcttgagccactgcgcctggccaaacatggaatttgttttatacagttgcaattatggtccattaatacaatctatttgtatgttatcagtaacagtaatactaacagtgaacccttattaagcatttactatgtgccaggcacaaggctaagagttttacagagatgatctcatttaccttgggttacttacccaaccaaggtttatagccagcaggtggcaaagcttgaattccaacccaactctgctgactcccaactacacccacctgcacacttgcctcttgggccttgtttgtctggcaagtcctaaatcccagactcatttgttcacttgcttgcttcctccctccctccctaccaaaacacagtatgatctgtcggttaaactcaatagactaaaaactccgggttcaaatgctagctcctccatcactagctgtatgaccttgggaaagtacttaatctctctgtgcctcaatttccatgtttataaaatgggataaagtgcccattatagtgcccatttcctaggattctatccaggagatgatgtgcctatttcctaaggttcttataatgagattctgcaaggacagcactccaaatagtacaggcacatggttttgacagttgtttctgttattattgaaataaaaagaacctatacctgttcccaggaagctcagagtctctcacaggccttttcagttcctggggctctcatatttcctcattctcccagactcctctgaccctactcttcctcaggttcttactgctcctgtgggaaatcagaaagagcagccagcagacaacaccaactgagatgaatgcagctgaaatggcacaggtcagtatggccaagaaacaccatgggctaatgttcagacccatggtatgaaagccagagtgggtgtgaatttcactcccatgtctcttatcttggatggttttcatctgcatgacccatttgcccaatgcccaatggatgtgaagatacagaaaagtccaggtactgttttcagggaagtaagatgtcctgtgccaactcttctcacttcagggtccaagtcagagtgcacaaggaaagcaggtggggctggcccaccagcaaaagcttcaggagagcaagggattggctgactgggctgcaagggtagtgttcaaagccagctgccttggaggccaagatagtggaggagctgcataaaacatggattttgcagccaagtaagagctggccttgattccagctcagccatttattagatgtgtggcattgggcaaatttacttaacctctctgaatatcagtttcctctgctgtaaaacaggctgtgaaactctcacttttttgacagttgggaggattaaatgtttgcaccccatagatacaaaacaaggaagggtgatttctccatctcttgtttgtggcggactgattataaagggcaagatgttttaaattttattttaaattttaaaaatatgtaagaatgctatgccttatactctaaggggttttgctcaaggtgtatcacttcctaataaaagtgcctaataaactgccgtttattgagtgctcaccctgagccagtacttatgctttacatgtataaatgcatttcaatcatcataataccctatccaacttccccattttatggatgagaaacctgaggttccacgaagtaagataacttgctcaaagtcacaaggctagccaatggcaggctgggatttgatcagcctgactctagcactcacactcctcaccactatgatggctctcaaaatgggcccctcagaccctctctgtattttgactctttggctttctcactcactaagctgtgagatccctatgagaaagaactggctccatcttagtctccactgtatccccaggacctaggaagtgcttggcacctagtagtggcttggaaagcacttgttaaatgaataaatgagtgatggtgtctctcttctctgtgcagcatatggtgaggggcccaccttcttacccctaaatggaagcaagcacatattctactaaaagcacaagcccattgctggggggctctagaagtgtttcagttatcatgtacttatgggaactgtagaagttggcgagacattttgctgagaccagttctgaaaaaaccaggccttcggacacgctgtcccaacactgccagtatcatttcaggggacttgcagctccatggaagctaacccccaggagaccagccagctggatttgactacctatagtcaccatccaggttgtcagatgccaattttttttcaggagaaccgctgaggctagccagaatatggctgggcagcaccctctaggctctcactggatagaacaggatacagagaaaggcctccctagccaccaagacctcttccttatagctgagaaacttccaaggatatgttaactatgaacaatgtttgtctgattaatttcaagtctgccagatgtatcagtgactaagaaaggaactgtggcctcagatcctgagtgaaatggttcatgcagaagtgactaatacagaagccaccaccccaaccccaaataaccacaagggctctgtgcagccatgtaaaacagaatcagtcaacaggaggctcacaagacaatcattcacctttgttccctgcagcaggtatcctgcaatctgagacttatcttgagctggggtaaggtctgaggcatgctggcagggtgtgtgagggttgggggtgagggtggtcacatccaggcaatcattctattaaggatgtgctagatgacccacagactcaggcctgactcctcaggagctcacagttagtaggggttcagacaagaacacaggtacataactaaaactctattgataagggcgcctcggtaaggtgctatgggaaccataaggatgcagttccatggcccagtcagctcatctggggaaaaataataaaacaaaaaggaagcagttccagacagaagaccatctccaaatggttctttattgaacacccactttggctaggcaatatcctccccctgccctctaatccaggctcaggtacccccagtggagtatcctcagaaggcaactcccaagaccaggagtaatgagagattgggcagagggtaagggacagcagggagacggaggaaaatgaagacaccagggaaagaggagaggcctgaactggacagctgatgctttgtcctgcccagcacccattcgtcccttcttcaggtaatatcatctgccaccacaaccaccagcaccaactctcagtctctgtgggtacatgccaggcctgtccatttggtgtattccatcttcctggccacaatgatgacttgaggctggataccttcctcgtctggaccaatgagaaccaaatccagcagttctgtcagcaaaggggagctctttttatcaataactggtgctgtggggccacactgtgaagcccaagaataaagccaactcaaatgaaagcagagctgagagccaaagagacagatccctgtttggagtcctgggatgcagcctgaagcccaatctagcccatccttttcagctacgtgagccattaaattccctctgccccaagtgaactggaaagagtcccaaccaaggtccttcccatctggttgttcttctggaagtattttgaggacaaggagattttcatctccagggttataaaagtaattgtgtggtgacaggctgttcctaggtccctggggtgagagccaccatggagacagagtccagctcgcctttcctaggatacacactcacgactgtcaacacatcttcgaatacatcagcacataattataaactcctattgtttgtagtagctattgtttttgtcttcccatcaccttgttttggatgaagaaaaggtcatgacccagactggattaatcatgtggccaaacatgcatggccacagtgactgatccaagaggacatggaactcacaacaaaccattgagaactttgggagtttccaaattcgaactggaagggaagaaacctttcattcagagcccccaagctaggaggatgcaggtctggagctatcagctgtcatggctccaaatgcacggcgaaggctcatgtgcagcaggaggaaaggaagccaacaaagaggcctggttgagtctgcttgttgtctcccaatggccattcttcccccactcctttttactagcagaatctccttcctcagagttttggctgcccaagtagaaactaaatttacagcctcctttgttgctaactgtggccacatggcaagacagtaggaacctgggtgcctgatgacatcatggaccagccccttgcctggcctggaccagctgactatcactgcactgttatgggagagagaaataaacttccatcttgtcgaagctatgtattttggtggttttatgtataaacattttaaaaataacaaactagaaaggagttctagatggaactagtggcaatgattacatacagctgttttgttttgcaaaccccacaactggatattaagtcaggatagctcctgctaaattctaacctcaaggctgaactgttctgccctattcacttacagatcagagcattaggcaaggacaaccttcttagcccctcacttctgaatcttccttctaagctaagaggtcagagcagaacgaggaaatgttgtgctatttggccagaaggagatggtaagaacagccctagtaacttcatttactcctgaggctctgtgcccacaaactgattctaagagcccttcctgtatatatgcgaattagctctaagtacagacattttggtgtgaattgtggagtttatggcaaatacagggtaggctgaatggttctaggccaggaagcaagagttcacaaatgcggtgtcttcaatgaaataaggtaagtaccttgaagcaaggagtaaccacctgactaatgcatccacatgagagactcaaatctaacacttggcaaaattacaatctgggatactgaggtccccacttttagtgaaagccaaaggccctaggtcaaaatgctaaaaagtcttttactaactatcctaggacagctaaggtcattttgggaagaagagagaaacactattcacccctcccttcaagttttaatagacaacaggaatctgggctctgaaaagtcacaaacacctttcccaagatgatgagcaactgcaacaactggccaaatgtgttagcagcagaaaagctgggcattacctgtgtgagaggcgctcagcatgggcagtgaatggccgtgagcagcgcaccagctacatagcctccacaccggaagggtgctgctgctctgcaggtccgtttcaggcgggatccagccatccacaggaccaaggggctggagtgttgggaacagatgattctgtgttccacagataatggtacaaagtgactgttcatagataaggtgtaagcacagcatttgaagacagctcctccagatggtctgtctgttagtgaattcttaagcacttagagccttgaagattgagaaattctaaagaaattttttaaaaggaggagggtggtagatgtcaaagacacaaaagctctttgtaggtgctgactggctcactttgtccccaggttcatcttagagctcaagcagattcaagacatgaggcagagatgctagacttgcgtcaggggcaaaaacttctggtagtagctcttggtgacgtcaatcatcagctcctgagtgcactccgggagctcccctgagaagagtcctgggcagcctgagaagacagtgaatggtggaaccacagtttctggaggtaatactgtgttgtcaagaattttgcagcagtctttcaacacacatcggcgcccaatcacacagttcttcccaacatgaacataggaaccaatctgtgctgcgttgaccacacaatcttcctcaataaagacatggtctccaatatgtaaaggaaagaatgcaacacctttgctgaacttcttgaatggtggccttatgacactacgacttttcacaacacaatgacgtccaactcttacatttgccagatcccctcggataatacagtcattcatcacaatggtctgcagtaatcccagctactcgggaggctgaggcaggagaatcgcttgaacctgggaggcggaggttgcagtgagccgagatcgcgccattgcactccagccttgccattgagaacgatgttctggcttccacacaacactgactggcgactgactttgttcccagatgccgtctcgatgtactcagacttgttgtagagcagctcgcccaactccatggccgccgcctccttccctcagccccggatcctgtcagagtcagtcggtcagtctttcagagattccggctacttcc

SEQ ID NO: 10983 - RNA, 9933 nt, Homo sapiens
  source 1..9933: mol_type = other RNA
ctgaatagctgggactacaggtgcacaccaccacacccagctaatttttttatttttgtagggactacaggtgcacaccaccacacccagctaatttttttatttttgtatttttacttttcaccatgtcggtcaggctggtctcaaactcctgacctcaggtgatctgcccacctcagcctcccaaagtgccgggattacaggcatgagccaccgtgcccagcccttaattgctgtctgaaccttttttttttttttcaacctgacctgaggcatcaattcaggcacagtataactctgaccagtaagcggaagctaacccaaatgctttccagggctgaggggacatcatgagagttgtggtcatgtacagaagcacagtcccaggggcacaggtggtacccctgtaaacaaagaatttgcaatattagggcacctcaagcaggacatccattaggctgtacaggtgaacagacctcctaccaggggaactcctgcccaagtgtttccagtcccatctgaaaagttcccagagtccttggcttccaagggactgcctgaaggcagtgagtcccaaacagttttgcttgttcaggatacaagttgatccatctcatgagcatggatgacatttgtgggagatcttcatggaaagcatagaagctagacccactctgttgtcagtctgaactcaaagcactcacagcacatggaaaggcagcactgggaattttccttcagcaagaggaggcttccagggatcaagcctccccaggtgccaggctttaattattttctccaatattacaaaaacagtcgtgccctgttcagcaatcataacattgcattttttcaaccatctcttactctcagctaggcctttcctctggaagggttgtatgtaagaggcacaaaagcatttttgtagataaacttttttttttttttttttgagatatggtctggctctgttgcccaggctagagtgcggtggcacgattttggctcactgcaacctccgcctcctgggctcaagccatcctcctacctcagcctcctaagtagctggaaccaaaggcacatgccatcatgtccagctaatttttgcattttttgtagacacaggatttcaccatgttgccaggctggtcttgaactcctgaactcaagcaatctgcccacctcggcctcccaaagtgctgggatcatatgcatccatcactgcgcctggccaacatttttttttttaactatcatcctagagttcaagtagataaacgtttttatgcaacttaaccagaaagacattcagaaattggtaattatgtgtggagggttgaattatgtccccacaaaaattcatgctgaagccctaaccatctacctgtacctcaaaatgtgagtatatttgaagataggccctgaagaggtaactaagttaaaatgggattgttaggatgggccctaatccaacctgagtggtatccttattaaaagagaagattaggacacagacacccagacagagggaccatacaaggacacagtaagaaggcagccatctgcaagccaagcagagaggcctcagaagaatctaaagctgtcgacaccttgtcctggactttcagcctccagaactgcaggaaaataagtttctattgtgtaagtcactcagtttgtggtactttgttatggtatccttagcaaactaataaaggatgaaaccctgaatttttaaaaatttcaaaatgtgtttacataatcttctaccccttttgtcctgattattcaatgagcagactagaaaagcctaatacctttctggggacagctacgttttaataatccacctaccttactaagctgtgtgtgctgggagaaaagtgagggaagtagagtcaggctgtcagtccactgttgcaagctgcaactaatcccaaaagctgaatgcaacaagtcaacagcagtgagagaagccccagagaaggtttgagtctggtctgtcaaaagcaggaggagaggtcatagtccttgcgatgtgcccttccccagcttggagcgtttggcaaatattagaagttaggaatgcaattagcctctgtattagagacaaagagcctatcagcagcttgatcttagatggtcccattagagaataagcccttttcagccaggttccaggacgttttcatagtttagcgctccacggagggggtccttaatctccaacggccccaacgtctgagtcctggtcattgagcctgtgcctgctttcagttcagcatagctcgtgttgaggctaaaacagctcaaggcagacagtagcaggtttcagcttagagtcagggccaggcaattaggatctgagaatttgagattctcaacaagcagctgcttttcttcagcagcagtgaaggcatgctgcatggccagacagctgtggtccaagtgacatgcaaggctgcctttttatcttgttggtcttagagtccaattgacccactcaaaaaaaatgcatattagactagacaatcatcagcctctaaggggagacatttgattttgacaagggttcattagcaatttaactgtattttcattttccaaacagattgcttctctttacatgttgtctccctctttcccgaggctccagtaagcacgaatcacagcaaaaataatcagttacagcctgttctggttccaatatccgaagaatttaaattccaacctatccactagtggcaaaaaactagaaagctgtatcccactaacacctttcatattttatttttgagtagctttatttgattagggtgatccctctagcatttatgaaattaacaagcataaaactttttttttaagagatgagtagctgggactacaggcgcacgccactgcgtccagctaaggtatgttttttaagcaatgaaatcaaccagtaaaaacaagttcaaatatttttcattcacacactcaaggcctgctgagcatccactgcatgtgttttacttgttccattagaaaggtttattaaaaaatggcggggcacagtggctcatgactgtaatcccagcacttagggaggccaagatcgcttgagcccaggagttcaagactagtctgggcaacatggtaaaaccctgtctctatttaaaaaataaacaaatacaagcaagtttttttttaaaaaatgatatattaaagaaaatcctcctaattctcttatgtcttttcatagctgtttccatgttctcatattcccatccttgtcaacatggaatttttgttgttgttgttgtggtttttttttttttttttgagacggagtctcgctctgtcgcccaggctggagtgcagtggcacaattacagctcactgcaagctccgccccctgggttcgcgccattctcctgcctcagcctcccaagtagctgggaatacaggcacccgccaccatgcctggctaatttttttgtatttttagtagagatggggtttcactgtgttagccaggatggtcttgatctcctgacctcgtgatctgcccacctcggcctcccgaagtgatgggattacaggcttgagccactgcgcctggccaaacatggaatttgttttatacagttgcaattatggtccattaatacaatctatttgtatgttatcagtaacagtaatactaacagtgaacccttattaagcatttactatgtgccaggcacaaggctaagagttttacagagatgatctcatttaccttgggttacttacccaaccaaggtttatagccagcaggtggcaaagcttgaattccaacccaactctgctgactcccaactacacccacctgcacacttgcctcttgggccttgtttgtctggcaagtcctaaatcccagactcatttgttcacttgcttgcttcctccctccctccctaccaaaacacagtatgatctgtcggttaaactcaatagactaaaaactccgggttcaaatgctagctcctccatcactagctgtatgaccttgggaaagtacttaatctctctgtgcctcaatttccatgtttataaaatgggataaagtgcccattatagtgcccatttcctaggattctatccaggagatgatgtgcctatttcctaaggttcttataatgagattctgcaaggacagcactccaaatagtacaggcacatggttttgacagttgtttctgttattattgaaataaaaagaacctatacctgttcccaggaagctcagagtctctcacaggccttttcagttcctggggctctcatatttcctcattctcccagactcctctgaccctactcttcctcaggttcttactgctcctgtgggaaatcagaaagagcagccagcagacaacaccaactgagatgaatgcagctgaaatggcacaggtcagtatggccaagaaacaccatgggctaatgttcagacccatggtatgaaagccagagtgggtgtgaatttcactcccatgtctcttatcttggatggttttcatctgcatgacccatttgcccaatgcccaatggatgtgaagatacagaaaagtccaggtactgttttcagggaagtaagatgtcctgtgccaactcttctcacttcagggtccaagtcagagtgcacaaggaaagcaggtggggctggcccaccagcaaaagcttcaggagagcaagggattggctgactgggctgcaagggtagtgttcaaagccagctgccttggaggccaagatagtggaggagctgcataaaacatggattttgcagccaagtaagagctggccttgattccagctcagccatttattagatgtgtggcattgggcaaatttacttaacctctctgaatatcagtttcctctgctgtaaaacaggctgtgaaactctcacttttttgacagttgggaggattaaatgtttgcaccccatagatacaaaacaaggaagggtgatttctccatctcttgtttgtggcggactgattataaagggcaagatgttttaaattttattttaaattttaaaaatatgtaagaatgctatgccttatactctaaggggttttgctcaaggtgtatcacttcctaataaaagtgcctaataaactgccgtttattgagtgctcaccctgagccagtacttatgctttacatgtataaatgcatttcaatcatcataataccctatccaacttccccattttatggatgagaaacctgaggttccacgaagtaagataacttgctcaaagtcacaaggctagccaatggcaggctgggatttgatcagcctgactctagcactcacactcctcaccactatgatggctctcaaaatgggcccctcagaccctctctgtattttgactctttggctttctcactcactaagctgtgagatccctatgagaaagaactggctccatcttagtctccactgtatccccaggacctaggaagtgcttggcacctagtagtggcttggaaagcacttgttaaatgaataaatgagtgatggtgtctctcttctctgtgcagcatatggtgaggggcccaccttcttacccctaaatggaagcaagcacatattctactaaaagcacaagcccattgctggggggctctagaagtgtttcagttatcatgtacttatgggaactgtagaagttggcgagacattttgctgagaccagttctgaaaaaaccaggccttcggacacgctgtcccaacactgccagtatcatttcaggggacttgcagctccatggaagctaacccccaggagaccagccagctggatttgactacctatagtcaccatccaggttgtcagatgccaattttttttcaggagaaccgctgaggctagccagaatatggctgggcagcaccctctaggctctcactggatagaacaggatacagagaaaggcctccctagccaccaagacctcttccttatagctgagaaacttccaaggatatgttaactatgaacaatgtttgtctgattaatttcaagtctgccagatgtatcagtgactaagaaaggaactgtggcctcagatcctgagtgaaatggttcatgcagaagtgactaatacagaagccaccaccccaaccccaaataaccacaagggctctgtgcagccatgtaaaacagaatcagtcaacaggaggctcacaagacaatcattcacctttgttccctgcagcaggtatcctgcaatctgagacttatcttgagctggggtaaggtctgaggcatgctggcagggtgtgtgagggttgggggtgagggtggtcacatccaggcaatcattctattaaggatgtgctagatgacccacagactcaggcctgactcctcaggagctcacagttagtaggggttcagacaagaacacaggtacataactaaaactctattgataagggcgcctcggtaaggtgctatgggaaccataaggatgcagttccatggcccagtcagctcatctggggaaaaataataaaacaaaaaggaagcagttccagacagaagaccatctccaaatggttctttattgaacacccactttggctaggcaatatcctccccctgccctctaatccaggctcaggtacccccagtggagtatcctcagaaggcaactcccaagaccaggagtaatgagagattgggcagagggtaagggacagcagggagacggaggaaaatgaagacaccagggaaagaggagaggcctgaactggacagctgatgctttgtcctgcccagcacccattcgtcccttcttcaggtaatatcatctgccaccacaaccaccagcaccaactctcagtctctgtgggtacatgccaggcctgtccatttggtgtattccatcttcctggccacaatgatgacttgaggctggataccttcctcgtctggaccaatgagaaccaaatccagcagttctgtcagcaaaggggagctctttttatcaataactggtgctgtggggccacactgtgaagcccaagaataaagccaactcaaatgaaagcagagctgagagccaaagagacagatccctgtttggagtcctgggatgcagcctgaagcccaatctagcccatccttttcagctacgtgagccattaaattccctctgccccaagtgaactggaaagagtcccaaccaaggtccttcccatctggttgttcttctggaagtattttgaggacaaggagattttcatctccagggttataaaagtaattgtgtggtgacaggctgttcctaggtccctggggtgagagccaccatggagacagagtccagctcgcctttcctaggatacacactcacgactgtcaacacatcttcgaatacatcagcacataattataaactcctattgtttgtagtagctattgtttttgtcttcccatcaccttgttttggatgaagaaaaggtcatgacccagactggattaatcatgtggccaaacatgcatggccacagtgactgatccaagaggacatggaactcacaacaaaccattgagaactttgggagtttccaaattcgaactggaagggaagaaacctttcattcagagcccccaagctaggaggatgcaggtctggagctatcagctgtcatggctccaaatgcacggcgaaggctcatgtgcagcaggaggaaaggaagccaacaaagaggcctggttgagtctgcttgttgtctcccaatggccattcttcccccactcctttttactagcagaatctccttcctcagagttttggctgcccaagtagaaactaaatttacagcctcctttgttgctaactgtggccacatggcaagacagtaggaacctgggtgcctgatgacatcatggaccagccccttgcctggcctggaccagctgactatcactgcactgttatgggagagagaaataaacttccatcttgtcgaagctatgtattttggtggttttatgtataaacattttaaaaataacaaactagaaaggagttctagatggaactagtggcaatgattacatacagctgttttgttttgcaaaccccacaactggatattaagtcaggatagctcctgctaaattctaacctcaaggctgaactgttctgccctattcacttacagatcagagcattaggcaaggacaaccttcttagcccctcacttctgaatcttccttctaagctaagaggtcagagcagaacgaggaaatgttgtgctatttggccagaaggagatggtaagaacagccctagtaacttcatttactcctgaggctctgtgcccacaaactgattctaagagcccttcctgtatatatgcgaattagctctaagtacagacattttggtgtgaattgtggagtttatggcaaatacagggtaggctgaatggttctaggccaggaagcaagagttcacaaatgcggtgtcttcaatgaaataaggtaagtaccttgaagcaaggagtaaccacctgactaatgcatccacatgagagactcaaatctaacacttggcaaaattacaatctgggatactgaggtccccacttttagtgaaagccaaaggccctaggtcaaaatgctaaaaagtcttttactaactatcctaggacagctaaggtcattttgggaagaagagagaaacactattcacccctcccttcaagttttaatagacaacaggaatctgggctctgaaaagtcacaaacacctttcccaagatgatgagcaactgcaacaactggccaaatgtgttagcagcagaaaagctgggcattacctgtgtgagaggcgctcagcatgggcagtgaatggccgtgagcagcgcaccagctacatagcctccacaccggaagggtgctgctgctctgcaggtccgtttcaggcgggatccagccatccacaggaccaaggggctggagtgttgggaacagatgattctgtgttccacagataatggtacaaagtgactgttcatagataaggtgtaagcacagcatttgaagacagctcctccagatggtctgtctgttagtgaattcttaagcacttagagccttgaagattgagaaattctaaagaaattttttaaaaggaggagggtggtagatgtcaaagacacaaaagctctttgtaggtgctgactggctcactttgtccccaggttcatcttagagctcaagcagattcaagacatgaggcagagatgctagacttgcgtcaggggcaaaaacttctggtagtagctcttggtgacgtcaatcatcagctcctgagtgcactccgggagctcccctgagaagagtcctgggcagcctgagaagacagtgaatggtggaaccacagtttctggaggtaatactgtgttgtcaagaattttgcagcagtctttcaacacacatcggcgcccaatcacacagttcttcccaacatgaacataggaaccaatctgtgctgcgttgaccacacaatcttcctcaataaagacatggtctccaatatgtaaaggaaagaatgcaacacctttgctgaacttcttgaatggtggccttatgacactacgacttttcacaacacaatgacgtccaactcttacatttgccagatcccctcggataatacagtcattcatcacaatggtcttgccattgagaacgatgttctggcttccacacaacactgactggcgactgactttgttcccagatgccgtctcgatgtactcagacttgttgtagagcagctcgcccaactccatggccgccgcctccttccctcagccccggatcctgtcagagtcagtcggtcagtctttcagagattccggctacttcc

SEQ ID NO: 10984 - RNA, 2161 nt, Homo sapiens
  source 1..2161: mol_type = other RNA
ctgaatagctgggactacaggtgcacaccaccacacccgactcatttttttttttttttttttttttttttttttttttttagtagagacagggtttcaccatgttggccaggtctcaaattcctgacctcaagcgatccttctgtctgggcctcccaaagttctgggattacctgcctgagtcacccgcccggccttaacagccataatttaaactagacagtatgggaacagctggagttagaaatcctagaaatcctgcttctgtaactgaccggtttacctctgacttgacttcaaacaggaagccctgaagattgaccttttcaagtacaacacttaaacaaagaactttccctctggaaggatttgtcggctacccttccaaaaacagacaggtgcggcctgacttcaagtgcaggccccgccctcctccggtgagtggccctagccctggaggcagctccatcagcctcagcatcccctcccggcgcccgcacgctcagaaaaaccacaggagcgggcgagcgggcgagcgggcgggcgggtgggcgggcggaggggagaggggatattttactccagcattcccttccacatttcgtattaaatacctgaaatatattaatcttaaaaaacaatatcgatacagtactcaatggatagaggcagtggagtgaacaagaagcccagattgcaaaatcgtaggtcataaaaaaactggagtgcgcgtgcgtcaggttccaggcacgcgagaaaaagcaacgcgaaagctttcagtctcggaggaggttttcgggcttggggtagccgaagagaacaaagtcggcctcgtagagtttatacagctgctgcctccaggccagggggatcttggcgaaccagtcctcctcccagctgctggcggtcctgttccggtagctcggggggaagcggagctgccggtccacctggagtagctgcagcagctgcgcggcgtcctcgtccagagtctccagcttccccacgaagtcgtagtcgatctggcacgggtggcagaggcggtacacctgccgccagtgctcgttgaagggcgccagcttctccgtgtgcgggtccagcaggtactggatgaagttggcgaaggacaccttgaggccagcgcggaaggcctcgcgcgccgaggcgggcaggctggtgtggttggcgtacagccgcagcatgggcacggcgaacttgcggtagaactcctcgttctccagctcgaacttgctgcggaaggcggagatcaggcgcacgaaggggtcgcgcacgaagaggaacttggtgtacttcttgagcttgaccttcatgaggtggcgggagagcttcccgtagcggcgccagaacttgttgaaggtcaggtgcgcgctggcgttgtgcacgtgctcgcgcgggatgcgcagcgggtcgcggtagggcgcaccgcggtgcagcaggcttccgctcagcacgatcatcacgcgcttccagttggtgcaggccaccttgggcacgtagcagtagatggccccgtgccggtcgtccacgatcaggtggctcagctccgagttggggatgtcgtcgaatgcgcgctccttggtggggaaggccaggctggagttggcgcagaagccccgcagcacgctcctccgctccgcctgctgccggccctggtctgggctgcgccgggcgtcgcgcggggaccagtcgtagcctctcacgctctcctccatgctccccggcgcaggcggctgctccgtctcctttctgggaaggtcgctctgcttcacgccagcactgagaaacttgtccagaaactcgtcgacatcggagtcggccgtgagctccctgtccctgtccggcccgggcgtgggcagcggcggccccgtgtgcggcctagagaaggacgtgtgcaagtagaagtgcgcggcgcctgcgctgtcccagtacacgatgatcagcaggatcatgaacaccgaccccagcaccagccacagccggaacagccgggccttggtcatcctgccccgggcgggctgggccctctccgggcctctcacttcagcttcctgcagagccggggcatcctgctgggaacctcgcgaccctcacctcgcgcccctcacctcgcgcccgcagccgccgccgccgccccgcgact

SEQ ID NO: 10985 - RNA, 2147 nt, Homo sapiens
  source 1..2147: mol_type = other RNA
ctgaatagctgggactacaggtgcacaccaccacacccgactcatttttttttttttttttttttttttttttttttttttagtagagacagggtttcaccatgttggccaggtctcaaattcctgacctcaagcgatccttctgtctgggcctcccaaagttctgggattacctgcctgagtcacccgcccggccttaacagccataatttaaactagacagtatgggaacagctggagttagaaatcctagaaatcctgcttctgtaactgaccggtttacctctgacttgacttcaaacaggaagccctgaagattgaccttttcaagtacaacacttaaacaaagaactttccctctggaaggatttgtcggctacccttccaaaaacagacaggtgcggcctgacttcaagtgcaggccccgccctcctccggtgagtggccctagccctggaggcagctccatcagcctcagcatcccctcccggcgcccgcacgctcagaaaaaccacaggagcgggcgagcgggcgagcgggcgggcgggtgggcgggcggaggggagaggggatattttactccagcattcccttccacatttcgtattaaatacctgaaatatattaatcttaaaaaacaatatcgatacagtactcaatggatagaggcagtggagtgaacaagaagcccagattgcaaaatcgtaggtcataaaaaaactggagtgcgcgtgcgtcaggttccaggcacgcgagaaaaagcaacgcgaaagctttcagtctcggaggaggttttcgggcttggggtagccgaagagaacaaagtcggcctcgtagagtttatacagctgctgcctccaggccagggggatcttggcgaaccagtcctcctcccagctgctggcggtcctgttccggtagctcggggggaagcggagctgccggtccacctggagtagctgcagcagctgcgcggcgtcctcgtccagagtctccagcttccccacgaagtcgtagtcgatctggcacgggtggcagaggcggtacacctgccgccagtgctcgttgaagggcgccagcttctccgtgtgcgggtccagcaggtactggatgaagttggcgaaggacaccttgaggccagcgcggaaggcctcgcgcgccgaggcgggcaggctggtgtggttggcgtacagccgcagcatgggcacggcgaacttgcggtagaactcctcgttctccagctcgaacttgctgcggaaggcggagatcaggcgcacgaaggggtcgcgcacgaagaggaacttggtgtacttcttgagcttgaccttcatgaggtggcgggagagcttcccgtagcggcgccagaacttgttgaaggtcaggtgcgcgctggcgttgtgcacgtgctcgcgcgggatgcgcagcgggtcgcggtagggcgcaccgcggtgcagcaggcttccgctcagcacgatcatcacgcgcttccagttggtgcaggccaccttgggcacgtagcagtagatggccccgtgccggtcgtccacgatcaggtggctcagctccgagttggggatgtcgtcgaatgcgcgctccttggtggggaaggccaggctggagttggcgcagaagccccgcagcacgctcctccgctccgcctgctgccggccctggtctgggctgcgccgggcgtcgcgcggggaccagtcgtagcctctcacgctctcctccatgctccccggcgcaggcggctgctccgtctcctttctgggaaggtcgctctgcttcacgccagcactgagaaacttgtccagaaactcgtcgacatcggagtcggccgtgagctccctgtccctgtccggcccgggcgtgggcagcggcggccccgtgtgcggcctagagaaggacgtgtgcaagtagaagtgcgcggcgcctgcgctgtcccagtacacgatgatcagcaggatcatgaacaccgaccccagcaccagccacagccggaacagccgggccttggtcatcctgccccgggcgggctgggccctctccgggcctctcacttcagcttcctgcagagccggggcatcctgctgggaacctcgcgcccctcacctcgcgcccgcagccgccgccgccgccccgcgact

SEQ ID NO: 10986 - RNA, 2133 nt, Homo sapiens
  source 1..2133: mol_type = other RNA
ctgaatagctgggactacaggtgcacaccaccacacccgactcatttttttttttttttttttttttttttttttttttttagtagagacagggtttcaccatgttggccaggtctcaaattcctgacctcaagcgatccttctgtctgggcctcccaaagttctgggattacctgcctgagtcacccgcccggccttaacagccataatttaaactagacagtatgggaacagctggagttagaaatcctagaaatcctgcttctgtaactgaccggtttacctctgacttgacttcaaacaggaagccctgaagattgaccttttcaagtacaacacttaaacaaagaactttccctctggaaggatttgtcggctacccttccaaaaacagacaggtgcggcctgacttcaagtgcaggccccgccctcctccggtgagtggccctagccctggaggcagctccatcagcctcagcatcccctcccggcgcccgcacgctcagaaaaaccacaggagcgggcgagcgggcgagcgggcgggcgggtgggcgggcggaggggagaggggatattttactccagcattcccttccacatttcgtattaaatacctgaaatatattaatcttaaaaaacaatatcgatacagtactcaatggatagaggcagtggagtgaacaagaagcccagattgcaaaatcgtaggtcataaaaaaactggagtgcgcgtgcgtcaggttccaggcacgcgagaaaaagcaacgcgaaagctttcagtctcggaggaggttttcgggcttggggtagccgaagagaacaaagtcggcctcgtagagtttatacagctgctgcctccaggccagggggatcttggcgaaccagtcctcctcccagctgctggcggtcctgttccggtagctcggggggaagcggagctgccggtccacctggagtagctgcagcagctgcgcggcgtcctcgtccagagtctccagcttccccacgaagtcgtagtcgatctggcacgggtggcagaggcggtacacctgccgccagtgctcgttgaagggcgccagcttctccgtgtgcgggtccagcaggtactggatgaagttggcgaaggacaccttgaggccagcgcggaaggcctcgcgcgccgaggcgggcaggctggtgtggttggcgtacagccgcagcatgggcacggcgaacttgcggtagaactcctcgttctccagctcgaacttgctgcggaaggcggagatcaggcgcacgaaggggtcgcgcacgaagaggaacttggtgtacttcttgagcttgaccttcatgaggtggcgggagagcttcccgtagcggcgccagaacttgttgaaggtcaggtgcgcgctggcgttgtgcacgtgctcgcgcgggatgcgcagcgggtcgcggtagggcgcaccgcggtgcagcaggcttccgctcagcacgatcatcacgcgcttccagttggtgcaggccaccttgggcacgtagcagtagatggccccgtgccggtcgtccacgatcaggtggctcagctccgagttggggatgtcgtcgaatgcgcgctccttggtggggaaggccaggctggagttggcgcagaagccccgcagcacgctcctccgctccgcctgctgccggccctggtctgggctgcgccgggcgtcgcgcggggaccagtcgtagcctctcacgctctcctccatgctccccggcgcaggcggctgctccgtctcctttctgggaaggtcgctctgcttcacgccagcactgagaaacttgtccagaaactcgtcgacatcggagtcggccgtgagctccctgtccctgtccggcccgggcgtgggcagcggcggccccgtgtgcggcctagagaaggacgtgtgcaagtagaagtgcgcggcgcctgcgctgtcccagtacacgatgatcagcaggatcatgaacaccgaccccagcaccagccacagccggaacagccgggccttggtcatcctgccccgggcgggctgggccctctccgggcctctcacttcagcttcctgcagagccggggcatcctgctgggaacctcgcgcccgcagccgccgccgccgccccgcgact

SEQ ID NO: 10987 - RNA, 4698 nt, Homo sapiens
  source 1..4698: mol_type = other RNA
ctgaatagctgggactacaggtgcacaccaccacacccggctaatttttgtatttttagtacagacagggtttcaccatgttggccaggctggtctcgaactcctgacctcaagtgatccacctgcctcagcctcccacagtactgggattatagatgtgagccaacgtgcctggccgaaactggtttattgaatgaactaagtccagaaagcgagggcttcatttttctctaaccattgccttacaacaaagttctgttggatctcctcccatcatcactcctgaatcttgggcagataccataaattttagtgacaaatctcactttagtcattgcacctctatttaagggattaaaatgtccaggccagtccaatttaacagcaatctcacacctcattcaaaaatctgcttggccttccttgcagtgaaatgacgaaggcatatagtcagtttctttactcttcctccattgtctctgtcttctctatattctagatgtccctatgccattgcaagggaagagggtattacacaaagaggagcagatcttcctgtagttaactattgaataaggcagacaggccagcatgatcctgccagctgctatggcagagtccaaatgctggctttttcatagggcacatctgtgagttattggagggccttgagtgtaccccacattgcacagttccatgatgcagggccacattatctggctgacctcttgcagcaacctccaccccaaacccctcttctgcctaaccccgtgtcctcttactgctatagtttctttgcacaacaggctaccctgttggctgatatcccgtcatgacaatgcaagcccagctactcttccatagtcaaagccatgtgaagaaattcacatccttttaccatgtcaataatgggagggcaggttgctatcagtgcttctcttctctcatcctgccattttgggtgctcaagccaacctttcacctcctgaattccccaggggggaagaactcatctattcattcaacaaatattcatcaagcacttgtatttgccaaacactatttaccagtctctgtgttcccagtgcccaccctcggactccagcaaacactcatcaagctcttccaagaattctcaagccacaccacatctgctgcactgaacctgtgtgctcctgttactctgcaagctttcagtcttggagtgggatgccaggctaccttctaccatgctgagtccctcacacttgtctgcaagaaattcaaagcaatctccctatggcctagaacctccgcttaatgactctttaatcacgcttttgactctagtcttctagagatggataatacggactgggagtcattggtctctttctgctcttttgataagtccagactggctgtgtctagtatcatgttggtgcagttactgtctttcgtcagctttgagcctttagccagaattctaagacaaccagaaaagtcccattcaatatccagctgcaaataaatttggccgagttttcttggaaagcaggtggatccacgtctttcacctcaacagcttatgattaagtccatatatccctttacatacatacactatcaagtcatgagtcctcattggttaattacatatttgtgtagcaggataaaaaattaaataagctattacacatatgtgaaacaaaagacttttttatatgccgtagctgatctaattttttccccaagccccagacttgaagagaatgatgacactgacccaaagaccaatatgattcacagggcactccgaggactggtgcatatgatgctgaagttgactgttcccttgctgccatgaagccatataaactcttgctcacaacagaatccatttgggaaagcagagtggagaggagctgaaaaactgagcatttactcaaaagagactgtttcaatttgaaacataatgattaaaccagaagagactgggctgtctctaactggcaggctaacctcaccgcctagctcagttccccagatgaaacattgtttttgttaagtctttcctgaaggcatgaggataatggaggcacctccagacagttacttacgactgtactattcaccatcatccaagtaaataatggtttcttaagttgaatttcctaaatttttttaagatttcacatcattgttttcagtgactagtgttaatttcatattaaaagcggctctaatgttagcccaaaagagcccacgtttgcttttctccttgggccactgcaaataagtccgctgcgtcatgagagccttcagcttgtggtacttgttgggaatgctgttctgtggaatgggttccagtaagatgaggattaagttattagatccttcatgaaagagattgtgatgggcaaaatagagttcgtaatggcaccactcactctggacaaagttgggagacaaaacaaagatggacttgtaactcttctcaatgcagttgatgatattttccacaatgctcttgccagggacaaagtttctctcatgaagacaaatctgtatatcttctttttctaggtaaggtaccaattcacttttcacccaggcagaatcatgttcactatatgaaataaaagcatgaaactggaggtttctttggagttcttctaagggtatgttcctggccctgcgccgagtctgggtccactggcacaccatcctgagataccagggcagatccaagtagatgcagagggaggtcacagtcacagccaacaccagcatggtggcaccgatggtgacgatcagcagagttatgttgcaggataattcagacatgtgaaagtcctttagtgggcttcctctataactttctgggtagtcacacttataagaatcaggccagccctctaacacttcacttgatacttggtctatatttttgacaaattctcttagctcacaggtacattggaatggattgtcccctgcttttattgacctcatcttctggcagctctggaagaaatcagccgatgggtgggaaactgaattgtgatcaatgatcaatacagaaaggctgctaaagctgccacatccaggaaggtcagttaaagaattgaaagcaacattgagttcttgcaaagcttccagttttacgacttgtttaggaacgctctttattttattgctgtgaagatcaagtaccttgatcctgggaggtaaacatctgaaaacagagtcagtaagcatatttgaagacaaatttaacaccactatactctcaacccaagtgcagttttctttatgtctaccagattccaaagaattccagctaacatccagtatttccaaagaaggcatatccttcgtcatgagacctactttgaaaaggtcttttaatccattcttttgtaagataagtgtctccaatttaactaacgtggaacatttttcaaaaatactatctgtgaaaacgttctgggtaaagttcaaaaacttgaatgtgcttggtgcatgaggacacagcatgtgtataaaaggtgtatctgaaatggttaacatcataatgttcatctcagaaaacacggtgtacaaagctgtctgtgaaaacagaaaaacttggttcgtgatatgttctattgtcaatgctttcaatgtcgttttagaataagtaaaatcttcttcacgaatgctttcaattattgttaaattgtaaatattgagatattccacaggtttgggccaaagaaattgaaagactctgaccaggcatttccaagtcgtttctatgtggttgagggtaaaattcagtaaggttgaacctctggtgagttctgataaaaatttaatgaaaacttgacagttgtcatcattcaatttaatattagtcagttgtaagcaccctaaagtattaactgatatgttcacttggatagcgaataaactagttgggtgaaaaacaaggtgaagggtttttgcattcagaatttgtagactttctgtctcattttcttttatataataatttcttaaatccagaaggatataacttagatgcaagtgagcaattggcagcaaatctaatttttgcagcttcatagcactcaatcccaagaaattcagttgtgataagttgccaaattccttacagatgggcagggccttgaaatcattgaatgagagatctaaatgcctgaaactcacaataggatggcaggatatcttttgcaactgattatgagataaatccaaatattctaaatcctggttgaacttgaaaacacttaaatcaagtagctggattctgttatgggaaagtctcaaaactgtcaactctgatagaaagctcatgtcagagacctgaagctcagcgatgtagttctgagacatatctaagactttggttttcagcggtaggtcttttggaacatgaataagacctctttttgacttgtctactgcaaattcatttccgtcggagaactggattctggttccaactattatgatcataaggcaaacaaaatggaagcttttaacaataggttctttgtctttggtcatgatgttgcagtggctatcctaaagggttgttcttcttcagagcatcttgatatgagtccaaattaatttggctaatgacaaagttggacatctccgtaagaatcacttctgctttcaggaggaagagaaaggctggcttcttgt

SEQ ID NO: 10988 - RNA, 4675 nt, Homo sapiens
  source 1..4675: mol_type = other RNA
ctgaatagctgggactacaggtgcacaccaccacacccggctaatttttgtatttttagtacagacagggtttcaccatgttggccaggctggtctcgaactcctgacctcaagtgatccacctgcctcagcctcccacagtactgggattatagatgtgagccaacgtgcctggccgaaactggtttattgaatgaactaagtccagaaagcgagggcttcatttttctctaaccattgccttacaacaaagttctgttggatctcctcccatcatcactcctgaatcttgggcagataccataaattttagtgacaaatctcactttagtcattgcacctctatttaagggattaaaatgtccaggccagtccaatttaacagcaatctcacacctcattcaaaaatctgcttggccttccttgcagtgaaatgacgaaggcatatagtcagtttctttactcttcctccattgtctctgtcttctctatattctagatgtccctatgccattgcaagggaagagggtattacacaaagaggagcagatcttcctgtagttaactattgaataaggcagacaggccagcatgatcctgccagctgctatggcagagtccaaatgctggctttttcatagggcacatctgtgagttattggagggccttgagtgtaccccacattgcacagttccatgatgcagggccacattatctggctgacctcttgcagcaacctccaccccaaacccctcttctgcctaaccccgtgtcctcttactgctatagtttctttgcacaacaggctaccctgttggctgatatcccgtcatgacaatgcaagcccagctactcttccatagtcaaagccatgtgaagaaattcacatccttttaccatgtcaataatgggagggcaggttgctatcagtgcttctcttctctcatcctgccattttgggtgctcaagccaacctttcacctcctgaattccccaggggggaagaactcatctattcattcaacaaatattcatcaagcacttgtatttgccaaacactatttaccagtctctgtgttcccagtgcccaccctcggactccagcaaacactcatcaagctcttccaagaattctcaagccacaccacatctgctgcactgaacctgtgtgctcctgttactctgcaagctttcagtcttggagtgggatgccaggctaccttctaccatgctgagtccctcacacttgtctgcaagaaattcaaagcaatctccctatggcctagaacctccgcttaatgactctttaatcacgcttttgactctagtcttctagagatggataatacggactgggagtcattggtctctttctgctcttttgataagtccagactggctgtgtctagtatcatgttggtgcagttactgtctttcgtcagctttgagcctttagccagaattctaagacaaccagaaaagtcccattcaatatccagctgcaaataaatttggccgagttttcttggaaagcaggtggatccacgtctttcacctcaacagcttatgattaagtccatatatccctttacatacatacactatcaagtcatgagtcctcattggttaattacatatttgtgtagcaggataaaaaattaaataagctattacacatatgtgaaacaaaagacttttttatatgccgtagctgatctaattttttccccaagccccagacttgaagagaatgatgacactgacccaaagaccaatatgattcacagggcactccgaggactggtgcatatgatgctgaagttgactgttcccttgctgccatgaagccatataaactcttgctcacaacagaatccatttgggaaagcagagtggagaggagctgaaaaactgagcatttactcaaaagagactgtttcaatttgaaacataatgattaaaccagaagagactgggctgtctctaactggcaggctaacctcaccgcctagctcagttccccagatgaaacattgtttttgttaagtctttcctgaaggcatgaggataatggaggcacctccagacagttacttacgactgtactattcaccatcatccaagtaaataatggtttcttaagttgaatttcctaaatttttttaagatttcacatcattgttttcagtgactagtgttaatttcatattaaaagcggctctaatgttagcccaaaagagcccacgtttgcttttctccttgggccactgcaaataagtccgctgcgtcatgagagccttcagcttgtggtacttgttgggaatgctgttctgtggaatgggttccagtaagatgaggattaagttattagatccttcatgaaagagattgtgatgggcaaaatagagttcgtaatggcaccactcactctggacaaagttgggagacaaaacaaagatggacttgtaactcttctcaatgcagttgatgatattttccacaatgctcttgccagggacaaagtttctctcatgaagacaaatctgtatatcttctttttctaggtaaggtaccaattcacttttcacccaggcagaatcatgttcactatatgaaataaaagcatgaaactggaggtttctttggagttcttctaagggtatgttcctggccctgcgccgagtctgggtccactggcacaccatcctgagataccagggcagatccaagtagatgcagagggaggtcacagtcacagccaacaccagcatggtggcaccgatggtgacgatcagcagagttatgttgcaggataattcagacatgtgaaagtcctttagtgggcttcctctataactttctgggtagtcacacttataagaatcaggccagccctctaacacttcacttgatacttggtctatatttttgacaaattctcttagctcacaggtacattggaatggattgtcccctgcttttattgacctcatcttctggcagctctggaagaaatcagccgatgggtgggaaactgaattgtgatcaatgatcaatacagaaaggctgctaaagctgccacatccaggaaggtcagttaaagaattgaaagcaacattgagttcttgcaaagcttccagttttacgacttgtttaggaacgctctttattttattgctgtgaagatcaagtaccttgatcctgggaggtaaacatctgaaaacagagtcagtaagcatatttgaagacaaatttaacaccactatactctcaacccaagtgcagttttctttatgtctaccagattccaaagaattccagctaacatccagtatttccaaagaaggcatatccttcgtcatgagacctactttgaaaaggtcttttaatccattcttttgtaagataagtgtctccaatttaactaacgtggaacatttttcaaaaatactatctgtgaaaacgttctgggtaaagttcaaaaacttgaatgtgcttggtgcatgaggacacagcatgtgtataaaaggtgtatctgaaatggttaacatcataatgttcatctcagaaaacacggtgtacaaagctgtctgtgaaaacagaaaaacttggttcgtgatatgttctattgtcaatgctttcaatgtcgttttagaataagtaaaatcttcttcacgaatgctttcaattattgttaaattgtaaatattgagatattccacaggtttgggccaaagaaattgaaagactctgaccaggcatttccaagtcgtttctatgtggttgagggtaaaattcagtaaggttgaacctctggtgagttctgataaaaatttaatgaaaacttgacagttgtcatcattcaatttaatattagtcagttgtaagcaccctaaagtattaactgatatgttcacttggatagcgaataaactagttgggtgaaaaacaaggtgaagggtttttgcattcagaatttgtagactttctgtctcattttcttttatataataatttcttaaatccagaaggatataacttagatgcaagtgagcaattggcagcaaatctaatttttgcagcttcatagcactcaatcccaagaaattcagttgtgataagttgccaaattccttacagatgggcagggccttgaaatcattgaatgagagatctaaatgcctgaaactcacaataggatggcaggatatcttttgcaactgattatgagataaatccaaatattctaaatcctggttgaacttgaaaacacttaaatcaagtagctggattctgttatgggaaagtctcaaaactgtcaactctgatagaaagctcatgtcagagacctgaagctcagcgatgtagttctgagacatatctaagactttggttttcagcggtaggtcttttggaacatgaataagacctctttttgacttgtctactgcaaattcatttccgtcggagaactggattctggttccaactattatgatcataaggcaaacaaaatggaagcttttaacaataggttctttgtctttggtcatgatgttgcagtggctatcctaaagggttgttcttcttcagagcatcttgatatgagtccaaattcaagatctctttttcagaagaagagaaaataacttgtaaatgaacggaaatacaatt

SEQ ID NO: 10989 - RNA, 5061 nt, Homo sapiens
  source 1..5061: mol_type = other RNA
ctgaatagctgggactacaggtgcacaccaccacacccggctaatttttgtatttttagtacagacagggtttcaccatgttggccaggctggtctcgaactcctgacctcaagtgatccacctgcctcagcctcccacagtactgggattatagatgtgagccaacgtgcctggccgaaactggtttattgaatgaactaagtccagaaagcgagggcttcatttttctctaaccattgccttacaacaaagttctgttggatctcctcccatcatcactcctgaatcttgggcagataccataaattttagtgacaaatctcactttagtcattgcacctctatttaagggattaaaatgtccaggccagtccaatttaacagcaatctcacacctcattcaaaaatctgcttggccttccttgcagtgaaatgacgaaggcatatagtcagtttctttactcttcctccattgtctctgtcttctctatattctagatgtccctatgccattgcaagggaagagggtattacacaaagaggagcagatcttcctgtagttaactattgaataaggcagacaggccagcatgatcctgccagctgctatggcagagtccaaatgctggctttttcatagggcacatctgtgagttattggagggccttgagtgtaccccacattgcacagttccatgatgcagggccacattatctggctgacctcttgcagcaacctccaccccaaacccctcttctgcctaaccccgtgtcctcttactgctatagtttctttgcacaacaggctaccctgttggctgatatcccgtcatgacaatgcaagcccagctactcttccatagtcaaagccatgtgaagaaattcacatccttttaccatgtcaataatgggagggcaggttgctatcagtgcttctcttctctcatcctgccattttgggtgctcaagccaacctttcacctcctgaattccccaggggggaagaactcatctattcattcaacaaatattcatcaagcacttgtatttgccaaacactatttaccagtctctgtgttcccagtgcccaccctcggactccagcaaacactcatcaagctcttccaagaattctcaagccacaccacatctgctgcactgaacctgtgtgctcctgttactctgcaagctttcagtcttggagtgggatgccaggctaccttctaccatgctgagtccctcacacttgtctgcaagaaattcaaagcaatctccctatggcctagaacctccgcttaatgactctttaatcacgcttttgactctagtcttctagagatggataatacggactgggagtcattggtctctttctgctcttttgataagtccagactggctgtgtctagtatcatgttggtgcagttactgtctttcgtcagctttgagcctttagccagaattctaagacaaccagaaaagtcccattcaatatccagctgcaaataaatttggccgagttttcttggaaagcaggtggatccacgtctttcacctcaacagcttatgattaagtccatatatccctttacatacatacactatcaagtcatgagtcctcattggttaattacatatttgtgtagcaggataaaaaattaaataagctattacacatatgtgaaacaaaagacttttttatatgccgtagctgatctaattttttccccaagccccagacttgaagagaatgatgacactgacccaaagaccaatatgattcacagggcactccgaggactggtgcatatgatgctgaagttgactgttcccttgctgccatgaagccatataaactcttgctcacaacagaatccatttgggaaagcagagtggagaggagctgaaaaactgagcatttactcaaaagagactgtttcaatttgaaacataatgattaaaccagaagagactgggctgtctctaactggcaggctaacctcaccgcctagctcagttccccagatgaaacattgtttttgttaagtctttcctgaaggcatgaggataatggaggcacctccagacagttacttacgactgtactattcaccatcatccaagtaaataatggtttcttaagttgaatttcctaaatttttttaagatttcacatcattgttttcagtgactagtgttaatttcatattaaaagcggctctaatgttagcccaaaagagcccacgtttgcttttctccttgggccactgcaaataagtccgctgcgtcatgagagccttcagcttgtggtacttgttgggaatgctgttctgtggaatgggttccagtaagatgaggattaagttattagatccttcatgaaagagattgtgatgggcaaaatagagttcgtaatggcaccactcactctggacaaagttgggagacaaaacaaagatggacttgtaactcttctcaatgcagttgatgatattttccacaatgctcttgccagggacaaagtttctctcatgaagacaaatctgtatatcttctttttctaggtaaggtaccaattcacttttcacccaggcagaatcatgttcactatatgaaataaaagcatgaaactggaggtttctttggagttcttctaagggtatgttcctggccctgcgccgagtctgggtccactggcacaccatcctgagataccagggcagatccaagtagatgcagagggaggtcacagtcacagccaacaccagcatggtggcaccgatggtgacgatcagcagagttatgttgcaggataattcagacatgtgaaagtcctttagtgggcttcctctataactttctgggtagtcacacttataagaatcaggccagccctctaacacttcacttgatacttggtctatatttttgacaaattctcttagctcacaggtacattggaatggattgtcccctgcttttattgacctcatcttctggcagctctggaagaaatcagccgatgggtgggaaactgaattgtgatcaatgatcaatacagaaaggctgctaaagctgccacatccaggaaggtcagttaaagaattgaaagcaacattgagttcttgcaaagcttccagttttacgacttgtttaggaacgctctttattttattgctgtgaagatcaagtaccttgatcctgggaggtaaacatctgaaaacagagtcagtaagcatatttgaagacaaatttaacaccactatactctcaacccaagtgcagttttctttatgtctaccagattccaaagaattccagctaacatccagtatttccaaagaaggcatatccttcgtcatgagacctactttgaaaaggtcttttaatccattcttttgtaagataagtgtctccaatttaactaacgtggaacatttttcaaaaatactatctgtgaaaacgttctgggtaaagttcaaaaacttgaatgtgcttggtgcatgaggacacagcatgtgtataaaaggtgtatctgaaatggttaacatcataatgttcatctcagaaaacacggtgtacaaagctgtctgtgaaaacagaaaaacttggttcgtgatatgttctattgtcaatgctttcaatgtcgttttagaataagtaaaatcttcttcacgaatgctttcaattattgttaaattgtaaatattgagatattccacaggtttgggccaaagaaattgaaagactctgaccaggcatttccaagtcgtttctatgtggttgagggtaaaattcagtaaggttgaacctctggtgagttctgataaaaatttaatgaaaacttgacagttgtcatcattcaatttaatattagtcagttgtaagcaccctaaagtattaactgatatgttcacttggatagcgaataaactagttgggtgaaaaacaaggtgaagggtttttgcattcagaatttgtagactttctgtctcattttcttttatataataatttcttaaatccagaaggatataacttagatgcaagtgagcaattggcagcaaatctaatttttgcagcttcatagcactcaatcccaagaaattcagttgtgataagttgccaaattccttacagatgggcagggccttgaaatcattgaatgagagatctaaatgcctgaaactcacaataggatggcaggatatcttttgcaactgattatgagataaatccaaatattctaaatcctggttgaacttgaaaacacttaaatcaagtagctggattctgttatgggaaagtctcaaaactgtcaactctgatagaaagctcatgtcagagacctgaagctcagcgatgtagttctgagacatatctaagactttggttttcagcggtaggtcttttggaacatgaataagacctctttttgacttgtctactgcaaattcatttccgtcggagaactggattctggttccaactattatgatcataaggcaaacaaaatggaagcttttaacaataggttctttgtctttggtcatgatgttgcagtggctatcctaaagggttgttcttcttcagagcatcttgatatgagtccaaattcgatatggacagcgactggaatactggtagcggtgttcatcaggaattgcagtttttatacacaatatatacaaagtatatatcggtcaaagtactagagagttgggcaacgataggagaagctactactttatactggttatatggtcaaaacaaatagttcacaatgaagatgtaacagataagaacagttatgcagcaagtaatattgcatcaaaatttacaaagtaaaaaatgttacaaaacacatggagacattgtgagtaaaagtatttagcatatttctctgggtcactgttagatcaagtagcaaaaaataaaaacatatatggaaatttgaatgagaaattaataaaggatttaatagagacataagctgtaccctacaaaaagagaacatcatatgtctaagtctctagagttcatagagcatttactaaaat

SEQ ID NO: 10990 - RNA, 4660 nt, Homo sapiens
  source 1..4660: mol_type = other RNA
ctgaatagctgggactacaggtgcacaccaccacacccggctaatttttgtatttttagtacagacagggtttcaccatgttggccaggctggtctcgaactcctgacctcaagtgatccacctgcctcagcctcccacagtactgggattatagatgtgagccaacgtgcctggccgaaactggtttattgaatgaactaagtccagaaagcgagggcttcatttttctctaaccattgccttacaacaaagttctgttggatctcctcccatcatcactcctgaatcttgggcagataccataaattttagtgacaaatctcactttagtcattgcacctctatttaagggattaaaatgtccaggccagtccaatttaacagcaatctcacacctcattcaaaaatctgcttggccttccttgcagtgaaatgacgaaggcatatagtcagtttctttactcttcctccattgtctctgtcttctctatattctagatgtccctatgccattgcaagggaagagggtattacacaaagaggagcagatcttcctgtagttaactattgaataaggcagacaggccagcatgatcctgccagctgctatggcagagtccaaatgctggctttttcatagggcacatctgtgagttattggagggccttgagtgtaccccacattgcacagttccatgatgcagggccacattatctggctgacctcttgcagcaacctccaccccaaacccctcttctgcctaaccccgtgtcctcttactgctatagtttctttgcacaacaggctaccctgttggctgatatcccgtcatgacaatgcaagcccagctactcttccatagtcaaagccatgtgaagaaattcacatccttttaccatgtcaataatgggagggcaggttgctatcagtgcttctcttctctcatcctgccattttgggtgctcaagccaacctttcacctcctgaattccccaggggggaagaactcatctattcattcaacaaatattcatcaagcacttgtatttgccaaacactatttaccagtctctgtgttcccagtgcccaccctcggactccagcaaacactcatcaagctcttccaagaattctcaagccacaccacatctgctgcactgaacctgtgtgctcctgttactctgcaagctttcagtcttggagtgggatgccaggctaccttctaccatgctgagtccctcacacttgtctgcaagaaattcaaagcaatctccctatggcctagaacctccgcttaatgactctttaatcacgcttttgactctagtcttctagagatggataatacggactgggagtcattggtctctttctgctcttttgataagtccagactggctgtgtctagtatcatgttggtgcagttactgtctttcgtcagctttgagcctttagccagaattctaagacaaccagaaaagtcccattcaatatccagctgcaaataaatttggccgagttttcttggaaagcaggtggatccacgtctttcacctcaacagcttatgattaagtccatatatccctttacatacatacactatcaagtcatgagtcctcattggttaattacatatttgtgtagcaggataaaaaattaaataagctattacacatatgtgaaacaaaagacttttttatatgccgtagctgatctaattttttccccaagccccagacttgaagagaatgatgacactgacccaaagaccaatatgattcacagggcactccgaggactggtgcatatgatgctgaagttgactgttcccttgctgccatgaagccatataaactcttgctcacaacagaatccatttgggaaagcagagtggagaggagctgaaaaactgagcatttactcaaaagagactgtttcaatttgaaacataatgattaaaccagaagagactgggctgtctctaactggcaggctaacctcaccgcctagctcagttccccagatgaaacattgtttttgttaagtctttcctgaaggcatgaggataatggaggcacctccagacagttacttacgactgtactattcaccatcatccaagtaaataatggtttcttaagttgaatttcctaaatttttttaagatttcacatcattgttttcagtgactagtgttaatttcatattaaaagcggctctaatgttagcccaaaagagcccacgtttgcttttctccttgggccactgcaaataagtccgctgcgtcatgagagccttcagcttgtggtacttgttgggaatgctgttctgtggaatgggttccagtaagatgaggattaagttattagatccttcatgaaagagattgtgatgggcaaaatagagttcgtaatggcaccactcactctggacaaagttgggagacaaaacaaagatggacttgtaactcttctcaatgcagttgatgatattttccacaatgctcttgccagggacaaagtttctctcatgaagacaaatctgtatatcttctttttctaggtaaggtaccaattcacttttcacccaggcagaatcatgttcactatatgaaataaaagcatgaaactggaggtttctttggagttcttctaagggtatgttcctggccctgcgccgagtctgggtccactggcacaccatcctgagataccagggcagatccaagtagatgcagagggaggtcacagtcacagccaacaccagcatggtggcaccgatggtgacgatcagcagagttatgttgcaggataattcagacatgtgaaagtcctttagtgggcttcctctataactttctgggtagtcacacttataagaatcaggccagccctctaacacttcacttgatacttggtctatatttttgacaaattctcttagctcacaggtacattggaatggattgtcccctgcttttattgacctcatcttctggcagctctggaagaaatcagccgatgggtgggaaactgaattgtgatcaatgatcaatacagaaaggctgctaaagctgccacatccaggaaggtcagttaaagaattgaaagcaacattgagttcttgcaaagcttccagttttacgacttgtttaggaacgctctttattttattgctgtgaagatcaagtaccttgatcctgggaggtaaacatctgaaaacagagtcagtaagcatatttgaagacaaatttaacaccactatactctcaacccaagtgcagttttctttatgtctaccagattccaaagaattccagctaacatccagtatttccaaagaaggcatatccttcgtcatgagacctactttgaaaaggtcttttaatccattcttttgtaagataagtgtctccaatttaactaacgtggaacatttttcaaaaatactatctgtgaaaacgttctgggtaaagttcaaaaacttgaatgtgcttggtgcatgaggacacagcatgtgtataaaaggtgtatctgaaatggttaacatcataatgttcatctcagaaaacacggtgtacaaagctgtctgtgaaaacagaaaaacttggttcgtgatatgttctattgtcaatgctttcaatgtcgttttagaataagtaaaatcttcttcacgaatgctttcaattattgttaaattgtaaatattgagatattccacaggtttgggccaaagaaattgaaagactctgaccaggcatttccaagtcgtttctatgtggttgagggtaaaattcagtaaggttgaacctctggtgagttctgataaaaatttaatgaaaacttgacagttgtcatcattcaatttaatattagtcagttgtaagcaccctaaagtattaactgatatgttcacttggatagcgaataaactagttgggtgaaaaacaaggtgaagggtttttgcattcagaatttgtagactttctgtctcattttcttttatataataatttcttaaatccagaaggatataacttagatgcaagtgagcaattggcagcaaatctaatttttgcagcttcatagcactcaatcccaagaaattcagttgtgataagttgccaaattccttacagatgggcagggccttgaaatcattgaatgagagatctaaatgcctgaaactcacaataggatggcaggatatcttttgcaactgattatgagataaatccaaatattctaaatcctggttgaacttgaaaacacttaaatcaagtagctggattctgttatgggaaagtctcaaaactgtcaactctgatagaaagctcatgtcagagacctgaagctcagcgatgtagttctgagacatatctaagactttggttttcagcggtaggtcttttggaacatgaataagacctctttttgacttgtctactgcaaattcatttccgtcggagaactggattctggttccaactattatgatcataaggcaaacaaaatggaagcttttaacaataggttctttgtctttggtcatgatgttgcagtggctatcctaaagggttgttcttcttcagagcatcttgatatgagtccaaattctctgtaatcctagcactttgggaggccgaggtggatggatt

SEQ ID NO: 10991 - RNA, 5119 nt, Homo sapiens
  source 1..5119: mol_type = other RNA
ctgaatagctgggactacaggtgcacaccaccacacccggctaatttttgtatttttagtacagacagggtttcaccatgttggccaggctggtctcgaactcctgacctcaagtgatccacctgcctcagcctcccacagtactgggattatagatgtgagccaacgtgcctggccgaaactggtttattgaatgaactaagtccagaaagcgagggcttcatttttctctaaccattgccttacaacaaagttctgttggatctcctcccatcatcactcctgaatcttgggcagataccataaattttagtgacaaatctcactttagtcattgcacctctatttaagggattaaaatgtccaggccagtccaatttaacagcaatctcacacctcattcaaaaatctgcttggccttccttgcagtgaaatgacgaaggcatatagtcagtttctttactcttcctccattgtctctgtcttctctatattctagatgtccctatgccattgcaagggaagagggtattacacaaagaggagcagatcttcctgtagttaactattgaataaggcagacaggccagcatgatcctgccagctgctatggcagagtccaaatgctggctttttcatagggcacatctgtgagttattggagggccttgagtgtaccccacattgcacagttccatgatgcagggccacattatctggctgacctcttgcagcaacctccaccccaaacccctcttctgcctaaccccgtgtcctcttactgctatagtttctttgcacaacaggctaccctgttggctgatatcccgtcatgacaatgcaagcccagctactcttccatagtcaaagccatgtgaagaaattcacatccttttaccatgtcaataatgggagggcaggttgctatcagtgcttctcttctctcatcctgccattttgggtgctcaagccaacctttcacctcctgaattccccaggggggaagaactcatctattcattcaacaaatattcatcaagcacttgtatttgccaaacactatttaccagtctctgtgttcccagtgcccaccctcggactccagcaaacactcatcaagctcttccaagaattctcaagccacaccacatctgctgcactgaacctgtgtgctcctgttactctgcaagctttcagtcttggagtgggatgccaggctaccttctaccatgctgagtccctcacacttgtctgcaagaaattcaaagcaatctccctatggcctagaacctccgcttaatgactctttaatcacgcttttgactctagtcttctagagatggataatacggactgggagtcattggtctctttctgctcttttgataagtccagactggctgtgtctagtatcatgttggtgcagttactgtctttcgtcagctttgagcctttagccagaattctaagacaaccagaaaagtcccattcaatatccagctgcaaataaatttggccgagttttcttggaaagcaggtggatccacgtctttcacctcaacagcttatgattaagtccatatatccctttacatacatacactatcaagtcatgagtcctcattggttaattacatatttgtgtagcaggataaaaaattaaataagctattacacatatgtgaaacaaaagacttttttatatgccgtagctgatctaattttttccccaagccccagacttgaagagaatgatgacactgacccaaagaccaatatgattcacagggcactccgaggactggtgcatatgatgctgaagttgactgttcccttgctgccatgaagccatataaactcttgctcacaacagaatccatttgggaaagcagagtggagaggagctgaaaaactgagcatttactcaaaagagactgtttcaatttgaaacataatgattaaaccagaagagactgggctgtctctaactggcaggctaacctcaccgcctagctcagttccccagatgaaacattgtttttgttaagtctttcctgaaggcatgaggataatggaggcacctccagacagttacttacgactgtactattcaccatcatccaagtaaataatggtttcttaagttgaatttcctaaatttttttaagatttcacatcattgttttcagtgactagtgttaatttcatattaaaagcggctctaatgttagcccaaaagagcccacgtttgcttttctccttgggccactgcaaataagtccgctgcgtcatgagagccttcagcttgtggtacttgttgggaatgctgttctgtggaatgggttccagtaagatgaggattaagttattagatccttcatgaaagagattgtgatgggcaaaatagagttcgtaatggcaccactcactctggacaaagttgggagacaaaacaaagatggacttgtaactcttctcaatgcagttgatgatattttccacaatgctcttgccagggacaaagtttctctcatgaagacaaatctgtatatcttctttttctaggtaaggtaccaattcacttttcacccaggcagaatcatgttcactatatgaaataaaagcatgaaactggaggtttctttggagttcttctaagggtatgttcctggccctgcgccgagtctgggtccactggcacaccatcctgagataccagggcagatccaagtagatgcagagggaggtcacagtcacagccaacaccagcatggtggcaccgatggtgacgatcagcagagttatgttgcaggataattcagacatgtgaaagtcctttagtgggcttcctctataactttctgggtagtcacacttataagaatcaggccagccctctaacacttcacttgatacttggtctatatttttgacaaattctcttagctcacaggtacattggaatggattgtcccctgcttttattgacctcatcttctggcagctctggaagaaatcagccgatgggtgggaaactgaattgtgatcaatgatcaatacagaaaggctgctaaagctgccacatccaggaaggtcagttaaagaattgaaagcaacattgagttcttgcaaagcttccagttttacgacttgtttaggaacgctctttattttattgctgtgaagatcaagtaccttgatcctgggaggtaaacatctgaaaacagagtcagtaagcatatttgaagacaaatttaacaccactatactctcaacccaagtgcagttttctttatgtctaccagattccaaagaattccagctaacatccagtatttccaaagaaggcatatccttcgtcatgagacctactttgaaaaggtcttttaatccattcttttgtaagataagtgtctccaatttaactaacgtggaacatttttcaaaaatactatctgtgaaaacgttctgggtaaagttcaaaaacttgaatgtgcttggtgcatgaggacacagcatgtgtataaaaggtgtatctgaaatggttaacatcataatgttcatctcagaaaacacggtgtacaaagctgtctgtgaaaacagaaaaacttggttcgtgatatgttctattgtcaatgctttcaatgtcgttttagaataagtaaaatcttcttcacgaatgctttcaattattgttaaattgtaaatattgagatattccacaggtttgggccaaagaaattgaaagactctgaccaggcatttccaagtcgtttctatgtggttgagggtaaaattcagtaaggttgaacctctggtgagttctgataaaaatttaatgaaaacttgacagttgtcatcattcaatttaatattagtcagttgtaagcaccctaaagtattaactgatatgttcacttggatagcgaataaactagttgggtgaaaaacaaggtgaagggtttttgcattcagaatttgtagactttctgtctcattttcttttatataataatttcttaaatccagaaggatataacttagatgcaagtgagcaattggcagcaaatctaatttttgcagcttcatagcactcaatcccaagaaattcagttgtgataagttgccaaattccttacagatgggcagggccttgaaatcattgaatgagagatctaaatgcctgaaactcacaataggatggcaggatatcttttgcaactgattatgagataaatccaaatattctaaatcctggttgaacttgaaaacacttaaatcaagtagctggattctgttatgggaaagtctcaaaactgtcaactctgatagaaagctcatgtcagagacctgaagctcagcgatgtagttctgagacatatctaagactttggttttcagcggtaggtcttttggaacatgaataagacctctttttgacttgtctactgcaaattcatttccgtcggagaactggattctggttccaactattatgatcataaggcaaacaaaatggaagcttttaacaataggttctttgtctttggtcatgatgttgcagtggctatcctaaagggttgttcttcttcagagcatcttgatatgagtccaaattctttctttggaagagtgaaaactctgagttggggaacttttattactgaatggcgtatggttaaaagctcttcactgatccatataacttctcccaactgcccatcagaacacccacagagacacacatacatttgaaaaatccacttggccactgaaaacaaagaagcacagaaatgtaatggcaggatccaggagcatcttcactcacaaaaatgtaactggaactgtgttagggcaaacctgccacactcaagctttgtctcaggaaaatagactccctgatgaaaggcagaaagaaatttgtcctctctctgtctctgattcaaacagtgaggatgagttccaactagtacttaatgagtagctaggcagtgtcccttttaccccaatggtactgacatgagtggatcagcatgctgagttttccttctacggactgccacactccattctccccaaactttacacttagtgatggacactaccaggtaagagctgg

SEQ ID NO: 10992 - RNA, 1487 nt, Homo sapiens
  source 1..1487: mol_type = other RNA
ctgaatagctgggactacaggtgcacaccaccacacctggctaattttttgtatttttagtagagatggggtttcaccttgttggccaggctggtctcgaactattgacctcaggtgatctgcccgccttggcctccctaagtgctgggattataggcgtgagccaccgtgcctggcctgcttggttaactttattcttccaactttaccagctgcattctcagtcatttaaaggatataggaatggaggccaaaacagaccatttggaggtcagggatgccatgttttctattggggcaatttcatggggcactgtgccttgtgaatgacagtgagtggaagacaaaggattctccatattattccaggatgggagcccattcgactgtaacactgtgcactttgaaagagctgaaactattccctaataccgggactcagctggcaacccaaggaagcactgttcatctgccacccaggcttggtgttaggacaggagaaagcaggcctgtgggctggaggccgtcacagggccgtcaatgcagacaaagggatgatctctcgagtctttgctgagccacatatggggaccacacatcacagtcttcactcctgcaaggtccacagtcccgtgcttctggagcacctccttatccctcctgttccaaaagcctctggcgtgtttccatcacaatctcctccattatttctggctttaagatgtctttgatctgatgtggaagggatgcttcatagcagtacaggatgctggtatcatacagcatcatcctctgagttaccagcgagatgatgcagttccgaagccgggatatcacctctcgatcagcaagagagacaggctccaggtttgcaatgaagccccctgcttcctcttctttgtgctcaggtgttgggtaaatccagatgaagccgttgttaccgagaatcactgaggcaccacatggcaaatcatgaaagtgggtcttctgccgtttcaccagggagggggaaacctggaccaaaaccccactgataaggtccccttcctgtaagaaacctctcattgcaagctcatcttctgcagatcttctcctcagctctcctccaggaaggttcatggacgagagcagcaagaccgaatccagcctggagttggtctccaccttccacctcttctgttgaacctctgtgattcgtcccactacgatgtctcctacttcaccaatgtatctggttttcaaagctttcacacagatcaacttgtttactctctccacagagccagcaacagatgcaatgagcttctcttctcccatatacgttccatggccccgcatgaatcctgtgtccgtagtgattgtatcccccggcaccactagatgtttcttagtgtcgcggcccagtctctcgctaagaggcttgcgagccactggaagcctcatctccatcgccatcttggcgccaatgagttgcgcaggcgcagctc

SEQ ID NO: 10993 - RNA, 2071 nt, Homo sapiens
  source 1..2071: mol_type = other RNA
ctgaatagctgggactacaggtgcacaccaccacacctggctaattttttgtatttttagtagagatggggtttcaccttgttggccaggctggtctcgaactattgacctcaggtgatctgcccgccttggcctccctaagtgctgggattataggcgtgagccaccgtgcctggcctgcttggttaactttattcttccaactttaccagctgcattctcagtcatttaaaggatataggaatggaggccaaaacagaccatttggaggtcagggatgccatgttttctattggggcaatttcatggggcactgtgccttgtgaatgacagtgagtggaagacaaaggattctccatattattccaggatgggagcccattcgactgtaacactgtgcactttgaaagagctgaaactattccctaataccgggactcagctggcaacccaaggaagcactgttcatctgccacccaggcttggtgttaggacaggagaaagcaggcctgtgggctggaggccgtcacagggccgtcaatgcagacaaagggatgatctctcgagtctttgctgagccacatatggggaccacacatcacagtcttcactcctgcaaggtccacagtcccgtgcttctggagcacctccttatccctcctgttccaaaagcctctggcgtgtttccatcacaatctcctccattatttctggctttaagatgtctttgatctgatgtggaagggatgcttcatagcagtacaggatgctggtatcatacagcatcatcctctgagttaccagcgagatgatgcagttccgaagccgggatatcacctctcgatcagcaagagagacaggctccaggtttgcaatgaagccccctgcttcctcttctttgtgctcaggtgttgggtaaatccagatgaagccgttgttaccgagaatcactgaggcaccacatggcaaatcatgaaagtgggtcttctgccgtttcaccagggagggggaaacctggaccaaaaccccctgacctagctaaagaaatatatcacgaagctaggtcactgcaagattggcgggatgaatgaaaaggagactacagaatatacatcctaagtatattcaaattggtgtccttcctgtttataattgctgtcgcctacatgcatacacatagtacacatttttgcagagaacgctttgggactcagaggctattcatacatcccagcagaaggtgaccttcaatactcttctctgtcatttccctttgcagtcttccttgcactctaagccagaactcatgtgccagacattagagaagctgaagccaatgaggaagtgagctggagcctcctgctggcccaggagcactgcgttgttccatgaccctagctcatacctgaaccccaaacactcatcttgcctgtgagatgtgtgcctctgggtaggtaaggagatgggtggagctgggtgcaaatccatgtctggtcctggcaggacagctcaagtccacgtcctgccaaggaagagtccgcaggacccagggttgtgaaagtcagcatactgcagcagtcctctgcctactccatgtacatcaacgtggctgtactgataaggtccccttcctgtaagaaacctctcattgcaagctcatcttctgcagatcttctcctcagctctcctccaggaaggttcatggacgagagcagcaagaccgaatccagcctggagttggtctccaccttccacctcttctgttgaacctctgtgattcgtcccactacgatgtctcctacttcaccaatgtatctggttttcaaagctttcacacagatcaacttgtttactctctccacagagccagcaacagatgcaatgagcttctcttctcccatatacgttccatggccccgcatgaatcctgtgtccgtagtgattgtatcccccggcaccactagatgtttcttagtgtcgcggcccagtctctcgctaagaggcttgcgagccactggaagcctcatctccatcgccatcttggcgccaatgagttgcgcaggcgcagctc

SEQ ID NO: 10994 - RNA, 2512 nt, Homo sapiens
  source 1..2512: mol_type = other RNA
ctgaatagctgggactacaggtgcacaccaccacacctggctaattttttgtatttttagtagagatggggtttcaccttgttggccaggctggtctcgaactattgacctcaggtgatctgcccgccttggcctccctaagtgctgggattataggcgtgagccaccgtgcctggcctgcttggttaactttattcttccaactttaccagctgcattctcagtcatttaaaggatataggaatggaggccaaaacagaccatttggaggtcagggatgccatgttttctattggggcaatttcatggggcactgtgccttgtgaatgacagtgagtggaagacaaaggattctccatattattccaggatgggagcccattcgactgtaacactgtgcactttgaaagagctgaaactattccctaataccgggactcagctggcaacccaaggaagcactgttcatctgccacccaggcttggtgttaggacaggagaaagcaggcctgtgggctggaggccgtcacagggccgtcaatgcagacaaagggatgatctctcgagtctttgctgagccacatatggggaccacacatcacagtcttcactcctgcaaggtccacagtcccgtgcttctggagcacctccttatccctcctgttccaaaagcctctggcgtgtttccatcacaatctcctccattatttctggctttaagatgtctttgatctgatgtggaagggatgcttcatagcagtacaggatgctggtatcatacagcatcatcctctgagttaccagcgagatgatgcagttccgaagccgggatatcacctctcgatcagcaagagagacaggctccaggtttgcaatgaagccccctgcttcctcttctttgtgctcaggtgttgggtaaatccagatgaagccgttgttaccgagaatcactgaggcaccacatggcaaatcatgaaagtgggtcttctgccgtttcaccagggagggggaaacctggaccaaaaccccctgacctagctaaagaaatatatcacgaagctaggtcactgcaagattggcgggatgaatgaaaaggagactacagaatatacatcctaagtatattcaaattggtgtccttcctgtttataattgctgtcgcctacatgcatacacatagtacacatttttgcagagaacgctttgggactcagaggctattcatacatcccagcagaaggtgaccttcaatactcttctctgtcatttccctttgcagtcttccttgcactctaagccagaactcatgtgccagacattagagaagctgaagccaatgaggaagtgagctggagcctcctgctggcccaggagcactgcgttgttccatgaccctagctcatacctgaaccccaaacactcatcttgcctgtgagatgtgtgcctctgggtaggtaaggagatgggtggagctgggtgcaaatccatgtctggtcctggcaggacagctcaagtccacgtcctgccaaggaagagtccgcaggacccagggttgtgaaagtcagcatactgcagcagtcctctgcctactccatgtacatcaacgtggctgtctgcagccactccattaagggaagaggtttttgttccactcagaaaataaaaacgttcacccagataaagctaagagactagtaaatcctaatttgttttaggaagtatgctctccttaaaatagtaaatagcttcaataatgcaacctcgtacaagaaaagcagtgaaattccatttagaggctcagatgacagagcaagctttgccagcaataacatccactggactgattggacgtttgtctaagggctgtttaaccagacccagcctgcctttgttcccaggacagcctcagccccagtgctgagctgcagcgccccctggaggaagagagacagctgcacctcccagcccacagttggaggggctcttctggtgaaagtcagtctccttggagaaaaaggataaaacttgttctttacaaggctactgacccatgaccctgtgaaccctgaccgtcactgataaggtccccttcctgtaagaaacctctcattgcaagctcatcttctgcagatcttctcctcagctctcctccaggaaggttcatggacgagagcagcaagaccgaatccagcctggagttggtctccaccttccacctcttctgttgaacctctgtgattcgtcccactacgatgtctcctacttcaccaatgtatctggttttcaaagctttcacacagatcaacttgtttactctctccacagagccagcaacagatgcaatgagcttctcttctcccatatacgttccatggccccgcatgaatcctgtgtccgtagtgattgtatcccccggcaccactagatgtttcttagtgtcgcggcccagtctctcgctaagaggcttgcgagccactggaagcctcatctccatcgccatcttggcgccaat

SEQ ID NO: 10995 - RNA, 2097 nt, Homo sapiens
  source 1..2097: mol_type = other RNA
ctgaatagctgggactacaggtgcacaccaccacacctggctaattttttgtatttttagtagagatggggtttcaccttgttggccaggctggtctcgaactattgacctcaggtgatctgcccgccttggcctccctaagtgctgggattataggcgtgagccaccgtgcctggcctgcttggttaactttattcttccaactttaccagctgcattctcagtcatttaaaggatataggaatggaggccaaaacagaccatttggaggtcagggatgccatgttttctattggggcaatttcatggggcactgtgccttgtgaatgacagtgagtggaagacaaaggattctccatattattccaggatgggagcccattcgactgtaacactgtgcactttgaaagagctgaaactattccctaataccgggactcagctggcaacccaaggaagcactgttcatctgccacccaggcttggtgttaggacaggagaaagcaggcctgtgggctggaggccgtcacagggccgtcaatgcagacaaagggatgatctctcgagtctttgctgagccacatatggggaccacacatcacagtcttcactcctgcaaggtccacagtcccgtgcttctggagcacctccttatccctcctgttccaaaagcctctggcgtgtttccatcacaatctcctccattatttctggctttaagatgtctttgatctgatgtggaagggatgcttcatagcagtacaggatgctggtatcatacagcatcatcctctgagttaccagcgagatgatgcagttccgaagccgggatatcacctctcgatcagcaagagagacaggctccaggtttgcaatgaagccccctgcttcctcttctttgtgctcaggtgttgggtaaatccagatgaagccgttgttaccgagaatcactgaggcaccacatggcaaatcatgaaagtgggtcttctgccgtttcaccagggagggggaaacctggaccaaaaccccctgacctagttttccatatttcaggctcctcgtgtgcaaagagacagctccgtcagagaacactgcctggacctcagcactgataaggtccccttcctgtaagaaacctctcattgcaagctcatcttctgcagatcttctcctcagctctcctccaggaaggttcatggacgagagcagcaagaccgaatccagcctggagttggtctccaccttccacctcttctgttgaacctataagccaagttccacacctggacacatgctccatgttcatgtgtcatatcataaataaccagtaaggccagatgtggtggctcacgcctgtaatcccagcactttgggaggccgaagctggtggatcacttgaggtcaggagtttgagaccagcctgaccaatataatgaaaccccatctctactaaaaatacaaaaattagctgggcgtggtggcgggtgcctgtaatcccagctacttgggaggctgaggcaggagaatcgcttgaacctgggaggtggaggttgcagtgagccaagatcatgccactgcactccagcctgggcgacagagcgagactccatctcaaaaaaaaaaaaacatgaaccagtaatctgaaatcgaacaagccacatatttacatcagaagccacacaacggccaaatgcaatgaatgcctttttcatgtaactacaagtggaatgactgtcccatgaatgaaatcgccagcctgcctcgactttgtaaacaccaatctgatatcgacgttacctctgtgattcgtcccactacgatgtctcctacttcaccaatgtatcttttgttctcacctggttttcaaagctttcacacagatcaacttgtttactctctccacagagccagcaacagatgcaatgagcttctcttctcccatatacgttccatggccccgcatgaatcctgtgtccgtagtgattgtatcccccggcaccactagatgtttcttagtgtcgcggcccagtctctcgctaagaggcttgcgagccactggaagcctcatctccatcgccatcttggcgccaatgagtt

SEQ ID NO: 10996 - RNA, 1545 nt, Homo sapiens
  source 1..1545: mol_type = other RNA
ctgaatagctgggactacaggtgcacaccaccacacctggctaattttttgtatttttagtagagatggggtttcaccttgttggccaggctggtctcgaactattgacctcaggtgatctgcccgccttggcctccctaagtgctgggattataggcgtgagccaccgtgcctggcctgcttggttaactttattcttccaactttaccagctgcattctcagtcatttaaaggatataggaatggaggccaaaacagaccatttggaggtcagggatgccatgttttctattggggcaatttcatggggcactgtgccttgtgaatgacagtgagtggaagacaaaggattctccatattattccaggatgggagcccattcgactgtaacactgtgcactttgaaagagctgaaactattccctaataccgggactcagctggcaacccaaggaagcactgttcatctgccacccaggcttggtgttaggacaggagaaagcaggcctgtgggctggaggccgtcacagggccgtcaatgcagacaaagggatgatctctcgagtctttgctgagccacatatggggaccacacatcacagtcttcactcctgcaaggtccacagtcccgtgcttctggagcacctccttatccctcctgttccaaaagcctctggcgtgtttccatcacaatctcctccattatttctggctttaagatgtctttgatctgatgtggaagggatgcttcatagcagtacaggatgctggtatcatacagcatcatcctctgagttaccagcgagatgatgcagttccgaagccgggatatcacctctcgatcagcaagagagacaggctccaggtttgcaatgaagccccctgcttcctcttctttgtgctcaggtgttgggtaaatccagatgaagccgttgttaccgagaatcactgaggcaccacatggcaaatcatgaaagtgggtcttctgccgtttcaccagggagggggaaacctggaccaaaaccccctgacctagttttccatatttcaggctcctcgtgtgcaaagagacagctccgtcagagaacactgcctggacctcagcactgataaggtccccttcctgtaagaaacctctcattgcaagctcatcttctgcagatcttctcctcagctctcctccaggaaggttcatggacgagagcagcaagaccgaatccagcctggagttggtctccaccttccacctcttctgttgaacctctgtgattcgtcccactacgatgtctcctacttcaccaatgtatctggttttcaaagctttcacacagatcaacttgtttactctctccacagagccagcaacagatgcaatgagcttctcttctcccatatacgttccatggccccgcatgaatcctgtgtccgtagtgattgtatcccccggcaccactagatgtttcttagtgtcgcggcccagtctctcgctaagaggcttgcgagccactggaagcctcatctccatcgccatcttggcgccaat

SEQ ID NO: 10997 - RNA, 1563 nt, Homo sapiens
  source 1..1563: mol_type = other RNA
ctgaatagctgggactacaggtgcacaccaccacacctggctaattttttgtatttttagtagagatggggtttcaccttgttggccaggctggtctcgaactattgacctcaggtgatctgcccgccttggcctccctaagtgctgggattataggcgtgagccaccgtgcctggcctgcttggttaactttattcttccaactttaccagctgcattctcagtcatttaaaggatataggaatggaggccaaaacagaccatttggaggtcagggatgccatgttttctattggggcaatttcatggggcactgtgccttgtgaatgacagtgagtggaagacaaaggattctccatattattccaggatgggagcccattcgactgtaacactgtgcactttgaaagagctgaaactattccctaataccgggactcagctggcaacccaaggaagcactgttcatctgccacccaggcttggtgttaggacaggagaaagcaggcctgtgggctggaggccgtcacagggccgtcaatgcagacaaagggatgatctctcgagtctttgctgagccacatatggggaccacacatcacagtcttcactcctgcaaggtccacagtcccgtgcttctggagcacctccttatccctcctgttccaaaagcctctggcgtgtttccatcacaatctcctccattatttctggctttaagatgtctttgatctgatgtggaagggatgcttcatagcagtacaggatgctggtatcatacagcatcatcctctgagttaccagcgagatgatgcagttccgaagccgggatatcacctctcgatcagcaagagagacaggctccaggtttgcaatgaagccccctgcttcctcttctttgtgctcaggtgttgggtaaatccagatgaagccgttgttaccgagaatcactgaggcaccacatggcaaatcatgaaagtgggtcttctgccgtttcaccagggagggggaaacctggaccaaaaccccctgacctagttttccatatttcaggctcctcgtgtgcaaagagacagctccgtcagagaacactgcctggacctcagcactgataaggtccccttcctgtaagaaacctctcattgcaagctcatcttctgcagatcttctcctcagctctcctccaggaaggttcatggacgagagcagcaagaccgaatccagcctggagttggtctccaccttccacctcttctgttgaacctctgtgattcgtcccactacgatgtctcctacttcaccaatgtatcttttgttctcacctggttttcaaagctttcacacagatcaacttgtttactctctccacagagccagcaacagatgcaatgagcttctcttctcccatatacgttccatggccccgcatgaatcctgtgtccgtagtgattgtatcccccggcaccactagatgtttcttagtgtcgcggcccagtctctcgctaagaggcttgcgagccactggaagcctcatctccatcgccatcttggcgccaatgagtt

SEQ ID NO: 10998 - RNA, 1475 nt, Homo sapiens
  source 1..1475: mol_type = other RNA
ctgaatagctgggactacaggtgcacaccaccacacctggctaattttttgtatttttagtagagatggggtttcaccttgttggccaggctggtctcgaactattgacctcaggtgatctgcccgccttggcctccctaagtgctgggattataggcgtgagccaccgtgcctggcctgcttggttaactttattcttccaactttaccagctgcattctcagtcatttaaaggatataggaatggaggccaaaacagaccatttggaggtcagggatgccatgttttctattggggcaatttcatggggcactgtgccttgtgaatgacagtgagtggaagacaaaggattctccatattattccaggatgggagcccattcgactgtaacactgtgcactttgaaagagctgaaactattccctaataccgggactcagctggcaacccaaggaagcactgttcatctgccacccaggcttggtgttaggacaggagaaagcaggcctgtgggctggaggccgtcacagggccgtcaatgcagacaaagggatgatctctcgagtctttgctgagccacatatggggaccacacatcacagtcttcactcctgcaaggtccacagtcccgtgcttctggagcacctccttatccctcctgttccaaaagcctctggcgtgtttccatcacaatctcctccattatttctggctttaagatgtctttgatctgatgtggaagggatgcttcatagcagtacaggatgctggtatcatacagcatcatcctctgagttaccagcgagatgatgcagttccgaagccgggatatcacctctcgatcagcaagagagacaggctccaggtttgcaatgaagccccctgcttcctcttctttgtgctcaggtgttgggtaaatccagatgaagccgttgttaccgagaatcactgaggcaccacatggcaaatcatgaaagtgggtcttctgccgtttcaccagggagggggaaacctggaccaaaaccccctgacctagttttccatatttcaggctcctcgtgtgcaaagagacagctccgtcagagaacactgcctggacctcagcactgataaggtccccttcctgtaagaaacctctcattgcaagctcatcttctgcagatcttctcctctctgtgattcgtcccactacgatgtctcctacttcaccaatgtatctggttttcaaagctttcacacagatcaacttgtttactctctccacagagccagcaacagatgcaatgagcttctcttctcccatatacgttccatggccccgcatgaatcctgtgtccgtagtgattgtatcccccggcaccactagatgtttcttagtgtcgcggcccagtctctcgctaagaggcttgcgagccactggaagcctcatctccatcgccatcttggcgccaatgagttgcgcaggcgcagctc

SEQ ID NO: 10999 - RNA, 1473 nt, Homo sapiens
  source 1..1473: mol_type = other RNA
ctgaatagctgggactacaggtgcacaccaccacacctggctaattttttgtatttttagtagagatggggtttcaccttgttggccaggctggtctcgaactattgacctcaggtgatctgcccgccttggcctccctaagtgctgggattataggcgtgagccaccgtgcctggcctgcttggttaactttattcttccaactttaccagctgcattctcagtcatttaaaggatataggaatggaggccaaaacagaccatttggaggtcagggatgccatgttttctattggggcaatttcatggggcactgtgccttgtgaatgacagtgagtggaagacaaaggattctccatattattccaggatgggagcccattcgactgtaacactgtgcactttgaaagagctgaaactattccctaataccgggactcagctggcaacccaaggaagcactgttcatctgccacccaggcttggtgttaggacaggagaaagcaggcctgtgggctggaggccgtcacagggccgtcaatgcagacaaagggatgatctctcgagtctttgctgagccacatatggggaccacacatcacagtcttcactcctgcaaggtccacagtcccgtgcttctggagcacctccttatccctcctgttccaaaagcctctggcgtgtttccatcacaatctcctccattatttctggctttaagatgtctttgatctgatgtggaagggatgcttcatagcagtacaggatgctggtatcatacagcatcatcctctgagttaccagcgagatgatgcagttccgaagccgggatatcacctctcgatcagcaagagagacaggctccaggtttgcaatgaagccccctgcttcctcttctttgtgctcaggtgttgggtaaatccagatgaagccgttgttaccgagaatcactgaggcaccacatggcaaatcatgaaagtgggtcttctgccgtttcaccagggagggggaaacctggaccaaaaccccctgacctagttttccatatttcaggctcctcgtgtgcaaagagacagctccgtcagagaacactgcctggacctcagcactgataaggtccccttcctgtaagaaacctctcattgcaagctcatcttctgcagatcttctcctctctgtgattcgtcccactacgatgtctcctacttcaccaatgtatcttttgttctcacctggttttcaaagctttcacacagatcaacttgtttactctctccacagagccagcaacagatgcaatgagcttctcttctcccatatacgttccatggccccgcatgaatcctgtgtccgtagtgattgtatcccccggcaccactagatgtttcttagtgtcgcggcccagtctctcgctaagaggcttgcgagccactggaagcctcatctccatcgccatcttggcgccaatgagtt

SEQ ID NO: 11000 - RNA, 1963 nt, Homo sapiens
  source 1..1963: mol_type = other RNA
ctgaatagctgggactacaggtgcacaccaccacacctggctttttttttttttttctttctttctaagtagagacagggtttcatcatgttggccaggatgatcccgaactcctgacttcagatgatccacctgcctcagactcccaaagtgctgggattacaggcgtgagccactgtgcccagcctcttggaaagatttggattcgcttcatggagccagggagcaggacataggtgaagaacccagcttgtggctcaagttggcctgaatagggttcgaggccctgctcccccgggcctctttgtccatgtgttcaaggaaaaaatgggagagtccaataccaaaaaggtggtcagagatccggagttgggcctgattccaaagaagggtcaaggccaaggcctcgagcttacgtgtggccaccagggggcagcagggatcggggtgtgcaggtggcctttcctccccgcctccactggcccatgggtcagaagtccagctcgggcatcagggtgtgcttgaccgggcagctgggggtctcgggttcctgctcgcagatgtccccggcaacacccatcctgtccccatccccattcccactcccgtccctgtgctctgcctcccaggctctctgctgggccggccagtccaggtgcgcccagcgggggtcagggcccccgatgacctcgtccaccaggtccgccaggtcgggcaggggctcgggtcgctccacaaggatgggcgcgaagggtcccaccagccagggcagcggcacggcctgcaccaccagctccagcagctcgtccacgcaggcgtgcgcgtgggccacgcgaccccggccctcggccagcgcggccgctggcacgtccctgaagcagcgggcatcagcgaaggcggtctgcagggcatccacactgcgccgcacctcagccaccttctcctgggcgccggcgggcaggccccgcacgctggactccagagcctctaccgtgccctgcagctcctgggtcaggctgcgggacagcaccagcgtctccagctctgcctggctccggcggcggctctccggagggcgctggccccattccccccacagctcgtgcaccttcccagggcaggccggggcggtgggggtcaccccacactgcatgtggtctatcagctccagcgtctcctgcagctgggccagggtgtcctgggcacggtgtttgctctgcctcagtttccccacagagtgctcgtaggccaggtggcggatccgtgctgacagggagccgaggcgcacaaagtagccctgctgtctcctctgatcctccaccgaacccacttcagggccttcagcctcagccgccagtgccgcgagctcttcctccgtcatgggcaggaagtgatccaccagctcctctgatttttccagtacaacatccacagcatggctcacggagcgcttcagctccacgctccagcgccggcccctccgggccaggtccaccacacccgtgacactgctggccaccacgtccttggctgaggtcaccaccgtctccgaaggttgctggagaaagggaagcttctcttccagcttgtccaggcccctgcaggcgaggctgttcatagtggccagctggggctgcaggtgctcgagcagcggctgggcgtggtccagggcacgggtggtcaggccgcacacgcagttctcagccaggcggcaggcggagcccagcagcgggtgcctgtccttggctgcactgtaaacatcgcagaccgcggtgcacgtggccctgaccaggggcagagccaccacacgctgcaccacgttctgctggtcctgctcccacacactggatctggggatctgagccgcctcttcttcagacatcgtgctgcaaacagggtcaccctgggcgcgagcggcttcagacaccagctgtctccgccgaccccaggctcgagtctccac

SEQ ID NO: 11001 - RNA, 12735 nt, Homo sapiens
  source 1..12735: mol_type = other RNA
ctgaatagctgggactacaggtgcacaccaccacactcggttaattttgtttgtttggaggcagggtttcaccatgttgtccaggctggtctcaaactcctgggctcaagcaatccaccggcctcagcctcccaaaatgctgagattacaggcatgagccaactgtgcccagccagccttagtatttatagacctggtttcctcaggtccaaatccctctccttcaatcaaatgttatacaactgcaactgtcctccacgtcgcctccatttatagagcattctatgaccttacctccccaccattaacttttccctggctaatttgaaactgcctgtacgagctttaaatgagttctttgtggacttcggaaagtgcttacattctcagcagttcctgtaatcctgtaaccaaagaagcgttgttgatggccaaggcttattcttcctacaaatatgattgagttctgacacctggtataatgttttctttaaaatgagagccaatgtaataaaattctttatggaatagtctgcaaaatgctttaatatattaataaaattaaaacaattttcacagaaaattttaataattttttctaacttcttttctgattgcacagttaattttaccatctagttacttcaataatattttctctgcctacagagcaaatataagggtaaattatacagaccctgctttagaaaggctcacaattcaagctggtctaacacgatgagtcaatgctatggaaaaacagaagagaccagttaattctattcagagtaagatcaaggaggacctcatatggatgaccttgggacttactggggtaactagaccgagaaggatgagtccattatcaggatttaagaatccagaactaagtgctaagtaaggggtttaaggaaagcatcagcaaaaattcactaattgttttcttttttttttttttttgagacggagtctcgctctgtctcccaggctggagtgcagtggcgcaatctcggctcactgcaagttgcgcctcccgggttcacgccattctcctgcctcaacctcccgagtagctgggactacaggcgcccgccaccacgcccggctaatttttttttttttatatttttagtagagacggggtttcaccgtgttagccaggatggtctcgatctcctgaccttgtgatccacctgcctcagcctcccaaagtgctgggattacaggcgtgacccaccgcgcccggcctcactaattgttagtttaaattaccacctacatgaagtcttataccctggctttgtattttatgttggctaaagagaatgattcaataagactataggataaaggcaccattaaaggtgcttcagtggcattctttcattgaggagaaatctgcagaagggtagcactttctagtaaaacatagtactctaaacacggttagcttacatgttcttccatttatttaagtgccttaaaaacaaaaggagaagcaaaaccctgaaagatcttggtttaattcttttcttctctaaaagtaggtttctgttttttggaggggatttaattgctcatctgatctgaatgcccatgaccagctcttgtttatcattggcatggccatgaacacaaacaatataaaatgccaatttaaccaatccaccatgcttgttttttcttttttcctaggaattaacagtggcaggccctggaaatagatgggtaagagcaaatctgtggtcatcaactaggtgcacagtccagtgggtgtgtgagatgcatgcacagggcagacagtagagcctgcaactgtgatggaattaacagggtaggccctgcaaacagatgagtaaaagcaaatctgcggccatcactaggtgcacagtgcagtgggggtgtgtgagatgcacagggcagacagtacagcctgcaactgtgatggaattaacagggtaggccctggaagatgagtaaaagcaaatctgcggccatcactaggtgcacagtgcagtgggggtgtgtgagatgcacagggcagacagtacagcctgcaactgtggcgcaggcgcagaacaggattgaatttcgctaaaaagacaaaggaagaaaaagtatggtctctgtcctcagggcattgcaacccattaggctgaatcatatgaactgcagattatgcaggtaaaatatggccacatatccacaccttcacagggctctgcctgacacacggaggacacaatcacaagagccaaagcagggaaggggcagggaaaaagtggacacaaccccaccccagtccagtggtgcggatcaataaatcgagacttacggccaatctgaaatagattctattcatgaaagtccttccagaaacaacattcaggatgacggcatcagtgttagccaagtgtctgagtggtctgggtgtcacatctgtgtgtgtgcccaaatggatgaaatttatgcacaaccaataagccccacaaaagtgattgttatgctgagccgaacaaccattttttacttccctttgtctctcccatagcttctctttccttttcacttcctggacctaccaaagccttggccttgggtggggaggcatccagtgactgtccttttcagcttcaacaatggcaacacaatctcttggctttgtatttgtgtaagagttccttttcacgatgagaatgtccaaaatagataccattctacattattcctttatttaaaaccacaggaaacatagaaacgagtttgaggaataccacttcaagatgggaatgggaggcaaaaataattcagccaactaggaggtgggcaaaatgctccgattccctttgttttcatatacgatttcattgaaggaagtggaagggatttaatagaaaagatatgatgatgacaaatcaagtcaatattgaaagaatactctaggcggggcgcagtggctcacgcctgtaatcccaacactttgggaggctgaggtgagcggatcacctgaggtcgggagttcgagaccagcctgaccaacacgaagaaaccccatctactaaaaatacaaaattagccgggtgtggtggcacatgcctgtaatcccagctacttgggagtctgaggcaggagaatcacttgaacccagtaggcggaagttgcggtgagccaagatcgtaccattgcactccagcctgggcaacaagactgaaactccgtctcaaaaaaaaaaaaaaaagtgtgtccaatcacagacttttgtcatttcttgagttctgaatcggctaaaacatccgagtgagttttctaacagtaaaagctgcatctctaggccactgaccacactgcagccctctgacagtgtcacactggcattattttgctgcttatggacaaaagaatgagcaatttcctgttggccagctctgaataccttattcactagaggctgagatggagtcagtactgctactacaggaacacgagtcaacatctcttaaatgctgtgtgccagactatgcgaagaaagggccttaaaaacattatctcatttaatcaccataagccttcgaagtagatgctagtattatccccatttcatagataactgaggagtggagaggtcagtcacctgcttcaagtcacagatcccataagtggcaaagtgagacagctggatgatccaacttcaaaagctgagcccccgcctgcttctatctgcttgatgcaaattcccaaaagtcaaaggcttctaaattcgcgctaattcctcaaatccctcctcttatcctggtgcagcctcagttggagtgacaggaagtttagatatgagtaagaaaacggaacctgacactgagttaaaaggacaatttcttccttcagagacaatcttactttatattaaacttcatttctgaagctccctgattctctaaaataatcaaaatgttcagcccaagatatgtcaaaatggtgaagaaatatcttaaaatccagttttcacccctctaacaataaagttaaatcctcccctttaatgggtctagtcagtggaagaacatttctctcattttaatcatttttctcctgatattttctctccttttaatcatttcttcacaaacatctgaatgtttatgctccaggcaagaggagagaaaatgatgagaatatccttatccctgggtgtgaggagtaattactctactgcccttttaaatacctttgaggtttatttcttaatttttttcctccaacttcagtttcacaacttcttcatgaaacaaggagcttggtaaaggaggccagcaagtaacaggttggctgtgagcgtgacatgaatgctcaggctgtaaactgtcttcctcagagagcagtgactccaatggtcagtgacatgcaggaggaaacgcaggattaggaccgactttccttaggtgtagcctcacgttttaatccctgaggtatgttgtaaatgggcagcgcatgaacaggtgatcaactcagaagacgagcttcataaaggttgccatagaactttagaatatgcctatggatggccaagtcacaaccagaattgagtccttaatcactgaccccatgtgtatttctatggaaggggagtgcagtatgtggcccaaaggttctgaaaaactgtgtgtgacagtctcctggctgtgtagcattttttgttgcttatagacaaaatttctctcctctatccaaatcagtaggccataggccattatttaagacaaacttttgagtataaaaaatttgtcttttacatacacaaatgcacacatatatagggtttgggacagactccacacccctaaaactagaggaaaaacaaggccctctagcaggtctgaacatgatgtaatcactttttcctttacttatgtaaaaggtaccctttgtcaaattagcacacttctggcaataattctggccccaaataaatagaaactttaagttgaaacttggcaattgtgaaatttccaaataattaaaaggtaaattttacagtaaagagactaatttttttctaattccatatgctataggctacaaaatatatatttaaattcccttaggtattaccaaatgtgtgttgaggtcctcaactggggttgagggaccctaactaggggttaatacatcatgcaaaattttccacgtattggaagaaacatcagaaatcagcttttgtgtgctccttaagccagttttaaaatagattttaaaatattcaccttccagctgattagcatgaaaggtttgaaaaatatacaaaagcagagtgctatggattgcatgtttatgtcctcccaaaattcatctgttgaaaccctaatctccaaagcaatggtattaggaggcggagctaataccataagtgggcctttgggaagtgagtaggtcctgagggtggagccctcatgaatattagcgccctcacaagaagggaaaggagagcttgcttgcttcctttctctctctctgccatgtaaggatgcaatgggaagatgatggctatcagcaaaccagggtaagggtgctcaccaggaactcaccttgatcttggacttcccagcctccagaacggtgagaaatttctgtcatttaagctacccagtgtatggtattttgttattgcagcctgagctgattaagacacagagtaactcacaaaataaataacatcaagtatcactggccaagccaatgagcagtcataccaaaagtagtttacttttaagatgtccatcttccacagaatctccaaggaagtagcttgcagtagtctcatccccacggaaatgatgcagtgattttatgcacaagggtaggagcaaaatgtgaactaatggtctacaaaactaatctcatctacaatagaagaaaacaagtcaggcctacttctccataccattcatgcctatggtggcaaaaggcagcatgagtctcatgctttgctggtgacattcaaatgtcagacagatttacttactcgagctctttggcggatgaaaagttttgtgtcaatacctcagggtttgctgcaatactaacaacctaaagaggaatgttcatggtcttccagggaaaaaattaaaaaaagaaagcccacaaaatagattctgaaatttcaggtttggtggggaaagaactgagagagaagcagagataggaaatggacaaatatatagactgaaatactacttaaggaggatacaggatttcttttaaaatacttgttctgaaagagatggtaccctcccccacctccgcccaagaggcagttctggaaatgtgagcatgttaggggtgccactgatgggcggccactactgagatttaacctgttggagcatgcgtgatacacaagccctgcagcttacagccctcacaacaaagagctgactcatcaacacaactttcaattgccccgcccaatattcatatagatgggaactcagtttacaataacaaatctatgatctcatttcattttatatataaacacacagaattttcagcccagttttaatatgctttggatttttcaagaatgcaatgagagaattctataaatggaaggaagcctatatactgagtgattatgagcaagaaagccagagccaggctgctttcattttaatcccagctctgccattattagcacataaccaggatgactagcacataacctgggtaactccctcatatgcaaaacgggactaacagcagtactcacctcatagatttattagaaaggtattagaacaatgccaggcacacagcaagcactatatgagtgaagccattacagactaggtatgcctagaactttatctaaagaattggccacattttagaaaatcatactgctgacatcgacccctttcctggtattgaactgccaatgcagcaggtctgaattggtaactaccacattcatggtgatttttcacatatttatatttatacacacacatacaaagtatgtgccctgcttagtagtttaattacatcttgtaatataaccatgctagaatatgtacatatgaaaataattatttcattataaaatatcttatctgtttcagttagaacgtcactgatgggtatgttttagaggctagttatattacctgctagtttcatttcagaatagtaaatggagtgatgtttttatgagtgaaggtaagcttcatcatccatgattttcatttgaagattgaaaagtgatgctataaaatattataataggggtaggtgttgagttgtgtctgggagagttttaacaatcactcttgtaaagtatcctgtcaaggagttcaagatcagcctggccaacatggtgaaactccatctctactaaaaatacaaaaattagccaggtgtggtggcgggcacctgtaatcccagctacttgggaggctgaggcaggagaattgcctgaacctgggaggcagaggctgcagtgagttgagattgtaccactgcactctagcctgggtgacagagtgagaatctgtctcagaaaaaaaaaaaaattttttttaaagaaataaaaataaagaatcctgtcaaaaagcatcatcaagcaacttcatatgtgaacacacgtccacaattaaacctggattactactgaggcaagcagtttccattaatttctaagaaatccatattaaactattatttatgtatgtccatagtagaggtttacaaaggttttttttttttagcagcaatatatttttcaaacacaattcaggagaaaacctcaaataaaaagaaagatgaagctgtggagggtgactgcaagtagaggagccaggaacttctctcgcgggtcctgggactccagggaacaaaggctgaaaagcaccaatctggttggccactgcctataatgaagactgactgccgaatattcacttaaaggatggctgttcaattcacaagtggcattttccccacagaaaaagagctcaccagccagctaaggcctccagagtgatttaactcatcatccagtggaactacagctcttagagttctccccacaatctggggagtaagaggagatgttgccacccacttcctgggcataaagccagctcaagacaagagtaaaacaggcagggctggctcgcccctcgtacacagctccctcctcatcaccagtgccctacacgagacctccccagcccacaccccaccctcctagtgtgttgaacaccctgtggtcacacactgcaagcctcttctctccatctgccaaacacccttgggtctccatgtctccatgaaataccagatctttttctttttgttttttttttgagacagagtctccttctgtcacccaggctggagtgcagtggcctgatcttggctcactacaacctccgcctccagggttcaagtgattctcctgcctcagcctcccgagtagctgggactacaggtgcccaccaccatgcgaagctgatttttagtagagacagggtttcaccatgttggccaggctggtcttgaactcctgaccccaggtaatccacccaccttggccccccaaagttctggaattacaggcatgagccactgcgccaggccgaaataccagatcttcatggcagttgtcttagaggtagagaagaaaacagccagactgagccgggtgtggtggctcatgcctgtaatcccagcactttgggaggctgaggccggcagatcagttgaggttgggagtttgagaccagcctggccaacgtagtgaaaccccgtctccactaaaaatacaaaaattagccaggcatggtggcgggcacctataatcccagctacatgggaggctgaggcaggagaatcgcttgaacctggaaggtggaggttgcagtgagctgagattgcgccactgcactccagcctgggtgacagattgagactccatctcaaaaacaaacaaacaaacaaaaaaaaccagcctgactgaattcagtcacagtaattatacatgagtggttgctagttcctttaaccacaccagaagcattttaaagggaagatgtttcctaactccagtgattttcatgggctgaattccaggcagttcagcaaactcaacaattccggtggtatgagaaagggcattttggagtaggagatttcggctctgcctaggaagatacctcagaaaattcccctcgtgcaatttcactttgcatatgcttctcctgttcttccatttctaatccataaaatcccaaaatgcttgggagggtttattttgattttttttaacaatactgccctgctggcaacagccacgatagtcacttgctcatctgaaaatgccttgcactttctttttcactagcttcgtgtatgacgcaaaacagaaatatttcaattacaggtgactaagagtaagaaaaatatacaactatatttaaaatacttaaattaacaagatagtacttttccattctaacaaaatatcatacattcagtttaaacaagagttaatatccagacacacgttttcaaaatacctgatgctagttgaaaattagtgaccatgaggctttccaagatatttctaattagcaaactgtgtacaattttgaagaagtgtacacaccgtgctggaagacagacactgaacaggtcaaaatgcaaactcatgtatctttcatcaacctaaatcttgttgcttcacttttctaaatgatactttggctgtcagcgaatcttatagcttcttttcccttaaagacaataatatataacaacaccaccccacacaaataaccataaacttctttgtgtgaaataagccctatcaaaatgtgttcatgtatttctgtaccaactgatctatactgagactgtcatgaaaaaggtatcaaacaagtgtaacaggcctacacttaaacctctgcctcaaaggagaaatcagatacttgccacgttattgcaaagtcaaagctgctacacttaaaatatggtagatagtttagaaaaatcaaatcaaaaatgttttctcactggctttttcagataaagaagttggaccacaaaccaacacatctgtgtgaaaacagccaccaatttgagtccccccagcccctcaaaaaggaacaatgccaccagtccctcacaatgaccataacgtctctggccaggactgcgatttctagcgcgtgtcttcacattctatctctggggaagcaagacaaacaggctctacccatttccctccttttgtctccacaagccagcacctaagatcctctgaatttgttcccatccaatcctgcaaacttccaagaagggcagtagataacttttcaaaagaaaaagaaattgcataaggtccctacataatactgaggctgaaacgagaagaggctgtccactgtaaaagcaaggcacttggggcaggagccaggcaggtggcctgagcagggtccctctcagtgagtcaacagtttgaggcgcgtaaaccagctgaccaggagggacggttctgtggacgaggacttcgtagctgaggagccagatttctttttggtcccttcctcctggaatggaatcgtggcgctgctgtggagatctgagttgatgtagcacctgcttcctcggatgtagtccgcaccccggaccagatgccgctcggtcgtgggtctggagaaccggtatgggggagaggagctctcttcaatgatcggaggaatccgctcgttactgaaataccggcaaagggcatcctcccctttcctgccatgacctcgaggtctggcaaaagggtccacaatccccatccagttcccatcagcaggcatggacaaaggccgtggcttgccataagatggtgttttctctctcatttttgtgggcagaatgttggtttccaccgagtacccaggcaactgatccgagtctgcaatggtgaatcttcgtctccggctttcctggtccaagaaggaattcggggactctgaacccttaggaccaggcaatggttgtttgcacttactggaccctccataaacaaaactgccattctcatcccggggagagtagggaacagcaggcggaggaggaatataaagatccaggatggctgacttctccttcttcagtgaggtatccatagtgctttcaggggactgggttgtcgcgggtggaggtgaggtctgtacaagaggtggcttccaccgtaggtttttcaggggagcaggagtaaagttgaaagacccggtggggcgcttcttaagcagtaacacaactccggtgggattctctctcaatttcttcaccagatttttcagctgccatcccaccacagtttgctgattaacttgaatgacttcgtcaccagcatgaatcttctgagatctgtctgcaggagaattttctgtggttccagtaatcacgtgtaacccatcataggttgatttgatgtacatgcccaggccttccccaggtttaatgtttggtaagtgaacttcctccagacatgcacactggctcatcacaggatctgtggtagatcggattgttttgtcacagatgccatttaaaaccttgaccacagttaaaactttatcctccatttccgctacaaagcaatccttctggactgtagtggtcaggtccaagcaaagctggataattttgttcttcgtgactgagaaatcagtgatccctgtaaacggagcccggtccagccacgccagcagggccttggcggcgccgatgagctccaccaccgaggtcaggaactcattgggggccttgcgggaggtgttgccatcgtaagcgggacttttccgtcggctacttatgtaattctgtaaattgtgggaagatgctctcagtttcagaaccaagttcttcatgttatcagtttcgaggccataattcagtgcacagagaaggtccacagcctccaacacaagctcctggtgtccaatccgtgtgacccccagctcctccaggtcctgatgggaaatctgcagcagctgctcgccgttgatcttctctcgttcaaacttgtggacatattgttgcaggcagtcatccaaccctctagtccagtccaccacttgtttggggctccacttggtcacgggttccatggtaaaccgcttcgcctctcgctgggctggagagtcgcagataaagtgctgctgcctgcgctccggtgccccttcccgggagggcgcgcccgcggctgctcccctgcgcccgagcgactccgtcaagactgcatggccgcggtcagccagtcgtcccagcgcggctccgccaggggagcccggccctctccctccagctgccacagtccagctgcagctcctccttcccccgccgccgccgggatcccgggcacagctgctgctcccgagcgacggcagctgcaggcacgccgggctgcgaccccagacccctggcctcggctcggcacgggagcctcccggcccgcgaccacttcctcggatctctcgaggcgcgatcggctctccctcggccggtcttctcgcctgctggctctccggggtccccgctccgcgtgcgctggcgtcccggagccttcccggcgcaggtcccacctcctgcgccgccctcccgtgccgccctggcagggccgagcgcagagcgtgcgcgctcgggttgcaaagtttcagctccggttgctgcaaaccgaat

SEQ ID NO: 11002 - RNA, 1340 nt, Homo sapiens
  source 1..1340: mol_type = other RNA
ctgaatagctgggactacaggtgcacaccaccacacttggctaatttttaaattttttgtagagaaaagatctcactatactgcccaggcaaattcttattagcaccaactgtcaccacaaactcatccttttctgacatacccattcaaaaaaactactaaccaaatgtccacaatcctgctaaaagtgttgaaaagctcttagtatagtattaagtgttatctacaaaatttgtgattaaccaaaacacacacaattgtgttcaaatgttatatatttgaagagtcaatttaacaattccttttggtagacttcttttgcacctctttacgcttcttttttttcctcttaccaccctctttgactcctgctgagaaaatagggggatctctgttgctggtaacccaagatatacctccctcatcattgtccacgaaagtatattgagatacatgtttggagctgtgagaatttggtgaatagttgttgaatgactgtgttctccagctgcattcttttgcaaagccctcttcattggccacactatttacaagaaaaaatgtcaactctccattatcttcagcttctctttcttgatcactttcaataattttctttgtattaatatttctgccattaacgattttgtctgaagttgtaacagatatgtagttgtccatcccactattatcaaaagccagggaagagaaagaagtaaggccttcatgccccaatgaaccctgtgatgtatatcctgtatcatatgaagaaaatttctcaaaaattggatattcactggcagtggagaaaaagtatcctgcatctctgtttctgtttccataggagcttcctggacgatttaacaggtcctcaagcgagtcttcaaagaagtgaaaagaaaatggatccctttcatgaaaaatttctttaaaaacatcatctggcttatggaatgtgaagccgtactcacattcatcatcaaaatgacttccacctccgtttaatccttctgtgccatatttatcataaatgtcccgtttctcatcatttgataatacctcgtatgcctcagctacttctttgaattttctctctgcttcttctttattttctggatttttatcagggtgccatttaagtgccactttatgataagcttttttaatgtcctcaggtgaagcatatctttgcagtcctagaacttcatagtaatccaccatgttttaacagatagttggaagtgggtgtgctgggtattgagaaccgtggtttcctcagctcaggctctgctggtggtggtgatagaggtagtgactgcaaataggtacacttttatgtt

SEQ ID NO: 11003 - RNA, 1744 nt, Homo sapiens
  source 1..1744: mol_type = other RNA
ctgaatagctgggactacaggtgcacaccaccacagctggataattttctgagtgccagtagtggcaacaactcaatcactaatattcagtgttgatggagcaagctgggtgtggtggcacgtgcctgtagtcccagctactcaggaggctgaggcaggagaatcacttgaaccagggaggcagaggctgcagtgagttgagattgcaccactgcattccagcctggacaacagagcgagactctgtctcaaaaaaaataaataaataaaaataaaaataaaaatttttacccttttgacagcatgtcaggcttctgggttctgttccccgagctcaaccctaagccaagcattttaaggtttgaggaaattaacttctcccagtttggaggaacattatagaagaagagataggagccattttaaatcatgaatgaaggaaggaaaaataccatagaaaagtctgggggtttgggtggtagaattggagaagctgacaatgtgaaagggagggaggaagggccagggcatctggaagtttcatttgaggggttcctgggagtttgtttctctagttttggggaatcattccctttgggcctgtctgatatgactgctgaaagagctgagtccattgtgcaatgcttgcaaaggtctagtaagaaggccatgctcttgtgcaaaagaaaatgagctgttttttcttccaaatctcagagtcaaaggagtcccagtgcttcagaacgcactccagaggaggggaaggggaagacagtgagggcgccacccctactgttttccctccttggttcctgggtcccagcatcttgttaaacatgcctcccatggttgcaggtgtgacccccagccatggaaccagaggaactaagtgattggggttagtcatgcttacccatgtgactctagtcctgcacttatgatttccttttgacttccaagacttgtgtgacctgtgtggctccctgaaaaatggatcttgggagagactatgtaacagttgcatttaggcaactgttgtatttccctccataatggaggaagtgtgctggtttgagctctatatcctgctattatgactcgtgctaaagtacccttagagaatggttccagttaacttccggacttaaattacccttactatttaagtactattttaattacaagcagaataggtgccttaaaaaaaacataggaaccaaatggctattttcctgctgatgggacagtattgagactaaaatttggttttggaggacattttcctccttattgttgaagacagagttttcccatttatggaagtagcataaagcctggtgtccagcagaggggtgcaaaaagggaggagaattgggaagccagagtgttttggcaaagggctgacaatgtgcctcatggagaggattcctatgccactgggtagggccgttgacctttaaatgccatgtgctctccagaccaagggcagagagagacctcactatggggagaggaggggaagacccactgttcctagaaaatcacaaaaatggcattgccttgagctctacctcagttactacggtatttcctgatcttgcctaacaggattacttccttgaactgtaaaaattcccactgcttcagaatgttctccccagcaagcctgtcccccaagtcttgtaaggctgccagccacactaatcatttttaaatagctgaagggggcccagtatttgatttg

SEQ ID NO: 11004 - RNA, 3317 nt, Homo sapiens
  source 1..3317: mol_type = other RNA
ctgaatagctgggactacaggtgcacaccaccacgccaggctaattgttgtgttttttactagagacagggtttcaccatgttgaccaggccggtctcgaactcctgacctcaggcgatctgcccacctcggcctctcaaagtgctgggattacaggcgtgaatcaccgcgcctggccaccaaccatgccaagctgatttttaaaaatattttggagagatgggggtctcactctgttgtctgggctggccttgaactctcaggctcaagcaactcagcctcccaaagtgctgggattaaaggcatgagccacagtgcccggtctgaagcacaggtgttttaaaggaaacctacagagcgttactcaaaaggaaatgaccattgtccaacgtcggggatgaagcagccattggtcggcgcgcacacgtccaggagtgcagggatgcaaaggcccgcaggtgggggaggtaggcggctcacacgagcccctctccgccccgccggccccgcttcttctcccctgcgccctcctctccctcgccaggtccccgttgcctcttccggaagcgggcccccagccggtgtctgggcggcaggagatccatgcccaggaccttgtgggtctgccggaaggccagcattcgcagggcgtgctgggcgctggcggtcacgtcttcccgctcttggagggtcatgggctcgagggcatctgtctggtctctctcgcagggatcctggagcccgggcccgtctgtcaggagcgtccctgtggccacgcactccaggactcgcctgactgcatccccggggcccaggggcccagccgcactgctcacagccttctccaccagcagctccatggcccaggctggcagggccccccaggtgggcacacgccggcagaggtccctcaggaccctgatgacgatcacgcatggctgcaggccgctggctcgagcctgaaaccacctggcatgacggagggcggccagggactcgaggcacttcttggggctcaggacatcacctgcatcagcctgaggctcctccacacctgggtctgtggaggggtcctcccgcatcagaggtgaggtgacagatatggtgacctgcatcctgggctcctcacaggaggagatgacaatgttggcttcagggtcggaggagacctcatactcatcctcggtcaccatctggagctgccggggcagctgctgggcgatcctccgcagcaggctgtgcgtgggcttctcggagcagagcagagcgaggcgcacgttcctgtccccacgcaggaggaggcctttcgccaggatgcctactcgcatgacgcctttcaggacccgagtctggggggcaacgctgctgcgcttgtcaccctcttcctctcggcggccccggtcctcctcggccagtgtgtcggacaccagcttgagggcccgctctgcgtgggacacggccctctgcacggccaggagctcctgctccgtggggtagatggtggcgtgcttgcacatgacgtgccggtcgtcgctggacgccggccgccgcccgggctggagtggggcgctggcgggtgactccggcctgcccatgagcagaggctgggcccagtcgggcggcgcgtggggcggcacgtcctggggtggctcctcctccagccgcctcctctccgcgtgccagcgccgcagctgctccagccgctcctccgccaggtgccgctgcttcctcatgcgctcctccaggaccttccgagcccggctgctgggctccgtggcaatgggaaggtccgggttcactttcttccggtactgcagccggtgccgccgccccctcacgtgcaggtccttcgcgttaaggtcgttgaaactgcactcgcacagcttgcagtggaagcgaagcactcgcccttcgtcgctgaacacctcctccacatattccgggcccaccggctgcgcatcagagcagcccgcgggagcttcctttgagcctccttgggtaggtgctccgggaccctctaatttaggttgggctggtttcccccactggggtctgcagcctgctgcctgtggctcaggaggcccctcgcataaggccttcgaggccacgggtctcttggccagcgctggcctgctcgaggcacacacgctggggccagtgggggacgtgggcttggcctctgccccgggggggctctctgtggccagtgcaggctcgagggtgggaatgggcttccccagtttggcgtgcagcttgaagaccttctggtgcttggatccccggatgtgggccgcgtaggcgtccgccccggtgcaggacacggcgcacaggtcgcaatgcagctgcgcctgcaccccgcgcgggctcccgttgggctgcacgcctgtcttctgggccgcctccttctttctgtgcttctgccctcccagatgttcccggtaggtctgggggccagcgcagctgatcttgcagatgtcgcagtagtgaagctggagctgcctgggccccgccttgggtctcggcagcttgctgggaagcggtggcttcgagtcggccctggggctgcttcctgagcctgcaggcgcgggcggcgggggcagctgctgcgggggtcccgggggaggcgggggctgcgctggaggatagaaagggctggcagcggagtacaccgacgcgtcatagttcgggtagcttggtgccgtgtaggcggtgcaggtggggttgtaggagggcggggggtaggaggtcacgatggaagctgacgactcgggctggacgcctgtcgccgtggggtaggtgtatcccgaggacaaggtgctcgctggctgtccggactccactatgggcgcctgctgtgggggctgagcgtggctgtgactgccatgggggctgggctgcccgcaggcttcttgggtccctggctggccggagtctgcggctgtcatgcgcccagactggagggcagcagactggaagtacggcctgtcctcatagctcctggcagctgctgactgtccgtagctgtaactgtcctggtaggtagccatggtggtggccgtggggacgggctcctggggtcggctgccgtaggcgaagtcctggccggagtggggctggtatccaccgtaccctgccggggcagctgggggaaaggccgggttcacggcagggtccatcccaggagtgggttgtgcagtatagctggcccccacagtgggcaggggaagggtcggaggctgggcgctgtactgcgggccgccgccctgcgcgaagtcgaaatactgactcgtcgccatcttggcgtcttccccgagcct

SEQ ID NO: 11005 - RNA, 534 nt, Homo sapiens
  source 1..534: mol_type = other RNA
ctgaatagctgggactacaggtgcacaccaccacgcctggctaatttttgtattttcagttagagacgtggttttaccatattggccaggctggtctcaaactcctgacctcgtgtgatccacccgcctgggcctctgaaagtgctgggattacaggtgtgagccaccaagcctggccgatccttttaagtttttaaaccagttaagctctttggttccccctcagagtcccaaggtcctgggtcactcaggatcacattttcctttaatcagttgtcactggtccccttttgtccctttgaacgtgctgtgggattagtagcagcatctggctgttggaaggactggctgggatctcaggtgaaataccctccctggccctccttacccttaagatctccctgaaaagtcagaccttgcttattggagtttgagatgcattctagtaaacccagacctaccagagagagggacccacgtctgaagaatcttccagcctggggaacctgtgactggccacacccttagcctaat

SEQ ID NO: 11006 - RNA, 1698 nt, Homo sapiens
  source 1..1698: mol_type = other RNA
ctgaatagctgggactacaggtgcacaccaccactcctggctaatttttgtatttttagtggagatggggtttcgccatgttggccaggctggtctcaaactcctaacctcaagtgatccactcgccttggcctcccaaagtgctgggattacagacgtgagccactgtgcctggccactcctgtacttttttaggggcccgtggaaaagaacactaagagacacagcagaggcccatgacccacacctaccatgggtactgggtatattgaacatcaatcaaaaaaacacattcaagatgtcaaggaaagttaaaaaaaaaaatcagtaataggaaacatttcaaagcaatggaattcaaaaaactggtctcacagcttaaaaagggacacaactgggatttaaaaagggtctggtaattcaggttctgccaaccttttgagaaatgtggcccctgacggccattgtagctgcttctgctcaggctcaagggcagcctcctgctgtaaggaatcaaagcttagataactgtccttactcaatttggtatttaaaagacgtcatcacattgtagtcctcttccaagtccagaacagtctcaacaatattatgatcatcaaaagcctgtttgaggctgccagggtcagcatctgtggccttctgagggctcttgtccatgagcagggcccaggcttcctctttgaagggtgaatcttggcaatgaccacacatgtggttcaattcgttttcaaattctatttttccagccaattcttcaatagttcggatgcttgtatggtcaatcatatcaagcagatcctttgtgacctcttggctagaattgttgagtggcatgtttgagtcagccttcaaatctctctccatatctttccttaaattttcttttctccagttttccccctctcctgcagttctccaagactctctttcaggtgccaaaatggaggaatgcatcaatacattttccttgctggttagaggttttctctcggggcacagagcatgtggttttgcatttaccggggcatggtttgttgcaaaggcagggttctcattctcaggagcacatgggacagcagcaaaaggagcagcagaagagcaggctgccagaggatgtcttctgcagaggagcctgtgcacgggcagcgagaaggagagcggcgcggcgctcagttccagcctctgctggcctgtgcactcctgggaataactaactccttcaaaggcccggtcaatggctgcagtcagttcctttctgcatcttcttagtttttcagacatttctcctaaaagcgaccatgtctttatgtaatgcattggaaatgcacaggacaacacaataatgttacaaatgaggctgcaaactacccctgaatggccacgatttcctggagcttggccctggctatagcaggacccacaaccctcgggctttcctcctggagtaggcggttctcggctctcgcggaggaacccgccatctgccagaagccccaaagacgccccgccccacttcccacagcttcctggcccgccccgccgctgcctcccgccccaccgcggctcccaggccgctggccctaccggcaccccccctttggcgagtcggcagccacgtccttgtcctcacccgcagcgcagtgacgccgacccatccaacggtcatcgcatgcgcgt

SEQ ID NO: 11007 - RNA, 4573 nt, Homo sapiens
  source 1..4573: mol_type = other RNA
ctgaatagctgggactacaggtgcacaccaccatacctggctaatttttgtatttttagtagagacggggttttggcatgttgtccaggctggtctcaaactcctgacctcaggtaatccacccgcctcggcctcccaaagtgctgggattaagggcgtgagacacagcgcccagcttttttttttttttttttaatgagacagggtctcagtctgtcacccaggctggagtgcagtggcacaatcatagctcactacatccttgaactcctgggctcaagtgatcctcccacctcagccttctgagtagctagaactgcaggtatataccacacctgctaactttttatttttttgtagagacagggtcttgaactcctagcctcaagtgatcctactgcctccacctcccaaagtgttgaaattaccggcctgagccactgtgtctggctcctatgttgtccttataagaacaccatgtgaagatacagagacacacagggaaaaagcccatgcgaagacagagacagagactgaagtgctgcagctacaagccaaagaatgctgaggattgctggcaaccaccagaagctaggggagaggcatgtgtggtttctgctgcagaccctccagaaggaactaaccctgctgacaacttgatttaggagtgctggcttcctgaattgtgagagaataaatttctgttctttaaagccaccaagtttgcagtagtttgttatggtagccctaggaaatacaggggcgttgggggaaatagggaaccattgctaatcagtacaaggtttctttttggggtgatgaaaatgttctaaaattgtggtgatggttgcgtaactctgtggatatattaaaaaccactgaataatacatttttttttttttttttttttttttagtcttgctctgttgcccaggctggggtgcagtggcttgatctcagctcactgcaacctctgcctgtcaggttcaagcaatcctcctgcctcagtctcctgaatagctgggattacaagtgcacaccaccaggcctggctaatttttgtatttttagtagagacggggtctcatcatgttggccagggtggtcttgaactgctgacctcaaatgatctacccaccttggcctcccaaagtgctgggattacaggcgtgagccactgtgcctggcctgaatagtatactttaaatggtgaattgtatggtatgtgaattatatctcaataaagctgtacattaaaaaaccctacacaaatagaaatatacctatcattatgtttttcctaattcctttttgatttaaacatttttagggtttaagactattataacctctatataaagaaaactgaaaattaagagacactggttcacaaattctaaaaacaaccattacctaaaatacttgaagaacaaactgagtggcctattttaagttaaaaaatatttaatattatcagataaaaacattgattgtgacagctttacatgtttcattccatacacagtgaaaaaggcaaagtattactaggaaggaaatgagtagttgggtttgtaaaagatttattgatcacataaaagcaatgaataggagatgacatatatctaactcatgattacaaaacttttagagacaactaggttaaatatttcatgttttggctaagggaaaagaattcatgatctcgttaaagaagttcaaagtcaacactgatattgtacaactaccagtgcttttctaatgatctagaaatttgctataaatagctttactttttgctagttaatcacttactatgattgggttttatttaacagtgaggactaaagaggcagaatccttttttaaccactggataaaacagagacataaattaatgatgggtgctaagctttacattttatgttaaaaagatggaatatatttaagtggattgaatatatttcatgaggagttggacatattaaacccccaaatctgtttaggaagttttgtgagaaagtgtgtatatgccttgactcactctggcttacttttaaaatggaatacatttggcactaaataaaataaatagacaagcaaactgtgagactaagctgctccatctgagttgcccatcttgacttacaattcatactatttcttagttcttgactgagcacaaacagacctaaccgtatagcacttctgtgatgcatgaaaatagaatctagagctaagatactgcgcttcactgatgagccaatcttctattctgccaaaatcatagttacaaatgtgaaattcattcaagaaattcacatttttaacaaatgcttatactttttcaagttttcttgctagatatgttcttggttttgtggccagctaaaatatgatctttgaattaaggaaatccatataaaagaaacatctattttataggaacctcatttcacttgaaactttctttaccaaaacaccaaaccaaaactttgtcaccaaactcctggaacaaagcactggtggctatattttagagtctctgatgagtctgaagtccactcatttttcatgtttcaagggtctcttcatttgctccacaagtatcgacaacacaaattaaacaacttgtgactggaaaagcacgaactttggagttggcaacccatttgtctgtttcggtattatattcgagaatgtgtcctaatcgaccaacaccctgaaaaccagccaagacataaactatagagccaactgctgcacatttcactgttacacccttccatggcattggtgagaccatcttccattcgttcaacttaatatcgtaatattccacattgtccagaccacctaaaccattctgaccacccacagcaaatatcttgtcttttacaaataccagcccatgattcttcctggcttcaatcattggacacagctcagtccatgtttctgtggcaggatcataaacttcacaggaattaagcactctcccagaaacattgtttcctaaacttccaccacaaacatagattaggccattggcttccaccatcccatggctgcagcgctgggtcagcatgctgggctttgtgtgccagctttcagttctcgtatcatagcactcaaataaatacagagctgagtttcctacttctgaacctccagatgtataaattttgccttctgcagcacatgcagcaaggctgtctcgaggtgtcggaggacccagtttcgaataccagctatccttcactacattatagcagtccattcgctttattgggaaaagctgagagcctcccaaaatgtatactacattgtcccaaaacacgcatgctgcatctcttcgtttttcaaaggggcagcggatgtctgtccagctataatcctttgggttaaaatatctacaagactgtggttgagagcctccaaatagggctatgcggtagtcatgtttctttcttctaggtcttgtgccatctacaagttcttctcggtcctctggagacagtagatggtacctcattccacttatcaccatcttaaggcattcaggattgtcttgaataagtggttcagcttgtaccgttttacttaagaaattctttgatataagaggaaacctgactttagcaaggatatcaaccataaatggctggcgattaggttcatcgtatttcaaccacctgactgcagcatcataaacctgatcctctgctctcacagtcagagtgtcctggttgagaagatgtgttactcgcttgacatcaagttgaagaaattcatcagttttgtaaacttcagtaaagtgctgatgaataaagtcatctgcagttgctttcaattcaggacaatctagacactccgctagcacacttataccaagacaatttgaagcatcaacttgttctttcaaaaaatcaacacacattttcttcacaggttcaatctgatattggtttgctgcatccagcaaagactgaacattgttgctattcacggaaattctagcagtataagcaaattccaccagttgttcaataatatcaggttcagcatctttgagttctacttcaaaggactttgattcaagcatgttagttgtgaacattaagttaaaaaaatgactggctgcagcaagaacaacacgatgagcaggtatctttctttcctggaccatgaggatcacgtcacacaacgttttctgtttccgcatgttattcatgacgcccatgaaacccgccaacaatttagcttcttcccgagcagcaagtttcttctcggtcttcttcttgctgctcttctccaccccagaggctgccatcctccctcagctcggttcacgcccggggctcgccgggccgggcgaggggtcgcactctctgggcacactggggattctatcgaccaaacacggcgatcggcagtgcagctgcagcgcccagctctggaacgcgcggcaggcggcggtggctcggccactgccgaaagacaaggccgggcggcccccttagaaacgctcagggagcgacgctaccaactgggctgcgtccccgggcagaaccc

SEQ ID NO: 11008 - RNA, 4704 nt, Homo sapiens
  source 1..4704: mol_type = other RNA
ctgaatagctgggactacaggtgcacaccaccatacctggctaatttttgtatttttagtagagacggggttttggcatgttgtccaggctggtctcaaactcctgacctcaggtaatccacccgcctcggcctcccaaagtgctgggattaagggcgtgagacacagcgcccagcttttttttttttttttttaatgagacagggtctcagtctgtcacccaggctggagtgcagtggcacaatcatagctcactacatccttgaactcctgggctcaagtgatcctcccacctcagccttctgagtagctagaactgcaggtatataccacacctgctaactttttatttttttgtagagacagggtcttgaactcctagcctcaagtgatcctactgcctccacctcccaaagtgttgaaattaccggcctgagccactgtgtctggctcctatgttgtccttataagaacaccatgtgaagatacagagacacacagggaaaaagcccatgcgaagacagagacagagactgaagtgctgcagctacaagccaaagaatgctgaggattgctggcaaccaccagaagctaggggagaggcatgtgtggtttctgctgcagaccctccagaaggaactaaccctgctgacaacttgatttaggagtgctggcttcctgaattgtgagagaataaatttctgttctttaaagccaccaagtttgcagtagtttgttatggtagccctaggaaatacaggggcgttgggggaaatagggaaccattgctaatcagtacaaggtttctttttggggtgatgaaaatgttctaaaattgtggtgatggttgcgtaactctgtggatatattaaaaaccactgaataatacatttttttttttttttttttttttttagtcttgctctgttgcccaggctggggtgcagtggcttgatctcagctcactgcaacctctgcctgtcaggttcaagcaatcctcctgcctcagtctcctgaatagctgggattacaagtgcacaccaccaggcctggctaatttttgtatttttagtagagacggggtctcatcatgttggccagggtggtcttgaactgctgacctcaaatgatctacccaccttggcctcccaaagtgctgggattacaggcgtgagccactgtgcctggcctgaatagtatactttaaatggtgaattgtatggtatgtgaattatatctcaataaagctgtacattaaaaaaccctacacaaatagaaatatacctatcattatgtttttcctaattcctttttgatttaaacatttttagggtttaagactattataacctctatataaagaaaactgaaaattaagagacactggttcacaaattctaaaaacaaccattacctaaaatacttgaagaacaaactgagtggcctattttaagttaaaaaatatttaatattatcagataaaaacattgattgtgacagctttacatgtttcattccatacacagtgaaaaaggcaaagtattactaggaaggaaatgagtagttgggtttgtaaaagatttattgatcacataaaagcaatgaataggagatgacatatatctaactcatgattacaaaacttttagagacaactaggttaaatatttcatgttttggctaagggaaaagaattcatgatctcgttaaagaagttcaaagtcaacactgatattgtacaactaccagtgcttttctaatgatctagaaatttgctataaatagctttactttttgctagttaatcacttactatgattgggttttatttaacagtgaggactaaagaggcagaatccttttttaaccactggataaaacagagacataaattaatgatgggtgctaagctttacattttatgttaaaaagatggaatatatttaagtggattgaatatatttcatgaggagttggacatattaaacccccaaatctgtttaggaagttttgtgagaaagtgtgtatatgccttgactcactctggcttacttttaaaatggaatacatttggcactaaataaaataaatagacaagcaaactgtgagactaagctgctccatctgagttgcccatcttgacttacaattcatactatttcttagttcttgactgagcacaaacagacctaaccgtatagcacttctgtgatgcatgaaaatagaatctagagctaagatactgcgcttcactgatgagccaatcttctattctgccaaaatcatagttacaaatgtgaaattcattcaagaaattcacatttttaacaaatgcttatactttttcaagttttcttgctagatatgttcttggttttgtggccagctaaaatatgatctttgaattaaggaaatccatataaaagaaacatctattttataggaacctcatttcacttgaaactttctttaccaaaacaccaaaccaaaactttgtcaccaaactcctggaacaaagcactggtggctatattttagagtctctgatgagtctgaagtccactcatttttcatgtttcaagggtctcttcatttgctccacaagtatcgacaacacaaattaaacaacttgtgactggaaaagcacgaactttggagttggcaacccatttgtctgtttcggtattatattcgagaatgtgtcctaatcgaccaacaccctgaaaaccagccaagacataaactatagagccaactgctgcacatttcactgttacacccttccatggcattggtgagaccatcttccattcgttcaacttaatatcgtaatattccacattgtccagaccacctaaaccattctgaccacccacagcaaatatcttgtcttttacaaataccagcccatgattcttcctggcttcaatcattggacacagctcagtccatgtttctgtggcaggatcataaacttcacaggaattaagcactctcccagaaacattgtttcctaaacttccaccacaaacatagattaggccattggcttccaccatcccatggctgcagcgctgggtcagcatgctgggctttgtgtgccagctttcagttctcgtatcatagcactcaaataaatacagagctgagtttcctacttctgaacctccagatgtataaattttgccttctgcagcacatgcagcaaggctgtctcgaggtgtcggaggacccagtttcgaataccagctatccttcactacattatagcagtccattcgctttattgggaaaagctgagagcctcccaaaatgtatactacattgtcccaaaacacgcatgctgcatctcttcgtttttcaaaggggcagcggatgtctgtccagctataatcctttgggttaaaatatctacaagactgtggttgagagcctccaaatagggctatgcggtagtcatgtttctttcttctaggtcttgtgccatctacaagttcttctcggtcctctggagacagtagatggtacctcattccacttatcaccatcttaaggcattcaggattgtcttgaataagtggttcagcttgtaccgttttacttaagaaattctttgatataagaggaaacctgactttagcaaggatatcaaccataaatggctggcgattaggttcatcgtatttcaaccacctgactgcagcatcataaacctgatcctctgctctcacagtcagagtgtcctggttgagaagatgtgttactcgcttgacatcaagttgaagaaattcatcagttttgtaaacttcagtaaagtgctgatgaataaagtcatctgcagttgctttcaattcaggacaatctagacactccgctagcacacttataccaagacaatttgaagcatcaacttgttctttcaaaaaatcaacacacattttcttcacaggttcaatctgatattggtttgctgcatccagcaaagactgaacattgttgctattcacggaaattctagcagtataagcaaattccaccagttgttcaataatatcaggttcagcatctttgagttctacttcaaaggactttgattcaagcatgttagttgtgaacattaagttaaaaaaatgactggctgcagcaagaacaacacgatgagcaggtatctttctttcctggaccatgaggatcacgtcacacaacgttttctttagatttatgtggcttgtcaagaaggttctgcaatcagtccctcccagcatgatatcaaattggcattgagtataaatccctgagcagattgtagattcaactacagctgggtggtagatttaaatcactgtttccgcatgttattcatgacgcccatgaaacccgccaacaatttagcttcttcccgagcagcaagtttcttctcggtcttcttcttgctgctcttctccaccccagaggctgccatcctccctcagctcggttcacgcccggggctcgccgggccgggcgaggggtcgcactctctgggcacactggggattctatcgaccaaacacggcgatcggcagtgcagctgcagcgcccagctctggaacgcgcggcaggcggcggtggctcggccactgccgaaagacaaggccgggcggcccccttagaaacgctcagggagcgacgctaccaactgggctgcgtccccgggcagaaccc

SEQ ID NO: 11009 - RNA, 4345 nt, Homo sapiens
  source 1..4345: mol_type = other RNA
ctgaatagctgggactacaggtgcacaccaccatacctggctaatttttgtatttttagtagagacggggttttggcatgttgtccaggctggtctcaaactcctgacctcaggtaatccacccgcctcggcctcccaaagtgctgggattaagggcgtgagacacagcgcccagcttttttttttttttttttaatgagacagggtctcagtctgtcacccaggctggagtgcagtggcacaatcatagctcactacatccttgaactcctgggctcaagtgatcctcccacctcagccttctgagtagctagaactgcaggtatataccacacctgctaactttttatttttttgtagagacagggtcttgaactcctagcctcaagtgatcctactgcctccacctcccaaagtgttgaaattaccggcctgagccactgtgtctggctcctatgttgtccttataagaacaccatgtgaagatacagagacacacagggaaaaagcccatgcgaagacagagacagagactgaagtgctgcagctacaagccaaagaatgctgaggattgctggcaaccaccagaagctaggggagaggcatgtgtggtttctgctgcagaccctccagaaggaactaaccctgctgacaacttgatttaggagtgctggcttcctgaattgtgagagaataaatttctgttctttaaagccaccaagtttgcagtagtttgttatggtagccctaggaaatacaggggcgttgggggaaatagggaaccattgctaatcagtacaaggtttctttttggggtgatgaaaatgttctaaaattgtggtgatggttgcgtaactctgtggatatattaaaaaccactgaataatacatttttttttttttttttttttttttagtcttgctctgttgcccaggctggggtgcagtggcttgatctcagctcactgcaacctctgcctgtcaggttcaagcaatcctcctgcctcagtctcctgaatagctgggattacaagtgcacaccaccaggcctggctaatttttgtatttttagtagagacggggtctcatcatgttggccagggtggtcttgaactgctgacctcaaatgatctacccaccttggcctcccaaagtgctgggattacaggcgtgagccactgtgcctggcctgaatagtatactttaaatggtgaattgtatggtatgtgaattatatctcaataaagctgtacattaaaaaaccctacacaaatagaaatatacctatcattatgtttttcctaattcctttttgatttaaacatttttagggtttaagactattataacctctatataaagaaaactgaaaattaagagacactggttcacaaattctaaaaacaaccattacctaaaatacttgaagaacaaactgagtggcctattttaagttaaaaaatatttaatattatcagataaaaacattgattgtgacagctttacatgtttcattccatacacagtgaaaaaggcaaagtattactaggaaggaaatgagtagttgggtttgtaaaagatttattgatcacataaaagcaatgaataggagatgacatatatctaactcatgattacaaaacttttagagacaactaggttaaatatttcatgttttggctaagggaaaagaattcatgatctcgttaaagaagttcaaagtcaacactgatattgtacaactaccagtgcttttctaatgatctagaaatttgctataaatagctttactttttgctagttaatcacttactatgattgggttttatttaacagtgaggactaaagaggcagaatccttttttaaccactggataaaacagagacataaattaatgatgggtgctaagctttacattttatgttaaaaagatggaatatatttaagtggattgaatatatttcatgaggagttggacatattaaacccccaaatctgtttaggaagttttgtgagaaagtgtgtatatgccttgactcactctggcttacttttaaaatggaatacatttggcactaaataaaataaatagacaagcaaactgtgagactaagctgctccatctgagttgcccatcttgacttacaattcatactatttcttagttcttgactgagcacaaacagacctaaccgtatagcacttctgtgatgcatgaaaatagaatctagagctaagatactgcgcttcactgatgagccaatcttctattctgccaaaatcatagttacaaatgtgaaattcattcaagaaattcacatttttaacaaatgcttatactttttcaagttttcttgctagatatgttcttggttttgtggccagctaaaatatgatctttgaattaaggaaatccatataaaagaaacatctattttataggaacctcatttcacttgaaactttctttaccaaaacaccaaaccaaaactttgtcaccaaactcctggaacaaagcactggtggctatattttagagtctctgatgagtctgaagtccactcatttttcatgtttcaagggtctcttcatttgctccacaagtatcgacaacacaaattaaacaacttgtgactggaaaagcacgaactttggagttggcaacccatttgtctgtttcggtattatattcgagaatgtgtcctaatcgaccaacaccctgaaaaccagccaagacataaactatagagccaactgctgcacatttcactgttacacccttccatggcattggtgagaccatcttccattcgttcaacttaatatcgtaatattccacattgtccagaccacctaaaccattctgaccacccacagcaaatatcttgtcttttacaaataccagcccatgattcttcctggcttcaatcattggacacagctcagtccatgtttctgtggcaggatcataaacttcacaggaattaagcactctcccagaaacattgtttcctaaacttccaccacaaacatagattaggccattggcttccaccatcccatggctgcagcgctgggtcagcatgctgggctttgtgtgccagctttcagttctcgtatcatagcactcaaataaatacagagctgagtttcctacttctgaacctccagatgtataaattttgccttctgcagcacatgcagcaaggctgtctcgaggtgtcggaggacccagtttcgaataccagctatccttcactacattatagcagtccattcgctttattgggaaaagctgagagcctcccaaaatgtatactacattgtcccaaaacacgcatgctgcatctcttcgtttttcaaaggggcagcggatgtctgtccagctataatcctttgggttaaaatatctacaagactgtggttgagagcctccaaatagggctatgcggtagtcatgtttctttcttctaggtcttgtgccatctacaagttcttctcggtcctctggagacagtagatggtacctcattccacttatcaccatcttaaggcattcaggattgtcttgaataagtggttcagcttgtaccgttttacttaagaaattctttgatataagaggaaacctgactttagcaaggatatcaaccataaatggctggcgattaggttcatcgtatttcaaccacctgactgcagcatcataaacctgatcctctgctctcacagtcagagtgtcctggttgagaagatgtgttactcgcttgacatcaagttgaagaaattcatcagttttgtaaacttcagtaaagtgctgatgaataaagtcatctgcagttgctttcaattcaggacaatctagacactccgctagcacacttataccaagacaatttgaagcatcaacttgttctttcaaaaaatcaacacacattttcttcacaggttcaatctgatattggtttgctgcatccagcaaagactgaacattgttgctattcacggaaattctagcagtataagcaaattccaccagttgttcaataatatcaggttcagcatctttgagttctacttcaaaggactttgattcaagcatgttagttgtgaacattaagttaaaaaaatgactggctgcagcaagaacaacacgatgagcaggtatctttctttcctggaccatgaggatcacgtcacacaacgttttctttcgccgatgtgctgcagaatttcacgaatgcaccacacaccaaggacagaacaaagagctcctcttaataacagaggcgcacagtgcccttagaagatggcatggtatttatcgatggctgcttctgctct

SEQ ID NO: 11010 - RNA, 2606 nt, Homo sapiens
  source 1..2606: mol_type = other RNA
ctgaatagctgggactacaggtgcacaccaccatgccagctaatttttgtatttttgatagagacagtttcaccatgttgcccaggcttgtctccaactcctgagctaaagcaacccaccggcctctgcctcccaaagtgctgggagccactgccaccactcccagcccccttcctttcttaagcactgttagggattgtgtctagctacctaaagaacatagactgactcttcccttaagccacttcccttgctgccaagttaggtcttcttccaataatataagatgctagaagacttagatcttgatcttatttctactttaaggttcgatagtccctcttaatgatttcctgtttagcttaatgcttggatgaggcggggcttcatgagctctatctttaagggtaaagccccttagccagacgtggtggtgcggcgtgcgcctgtagtcccagctattcggaaggttgaggcaggagaattgcttgagcctgggaggcggagattacggtgagccaagatcacaccactgcactccagcctgggcaacagaccaagaccttgtctccaaaaaaaaaaaaaaaaaaaggtaatgccgctttatctactaaggctaggcattattccatgccaaatattaccttctatgttcctaggttgctggttacttcagaccataatccctccatgacccacctaaggctgtccatgggactctgcctaatgctgctaatcctggtgggtgtaatgggaaccacagcctaccagaaaagagccactcttcctgtgagaccatctgcctcttaccattcaccagagctccacagcacaagggtcccagttagaggaataagggaggtgtgatgttgcccagaacatgacagggggtaaggaagagaataatttcttgtgagacaactggatggaaaatctattgtgtatacttaatttctactttctttggaatgcctctttccccggttgtcaatattatatagcctggcaatgaaaaaagggtgaagttttacagttctaaagatccattctttattttggtacaaaaataaattgttcaacctgtaaattgtcacttattttcgtattgttgtaaagcaaacttacagaataggaacacctgctaccagttccaagaatatcacatacatatgccttagaaaaaggccaggtatgatggttcatgcctgtaatcccagcactttgggaggccaaggtgagaatggatcgcttgaggccagcagttcaagaccagactagaaaacgtagcatgacccctgtatctacagaataatttaaaaattagccagatattgttgtgcgggcctgtagtcctagatactcaggagactgaggcagaaagattacttcagcctagaatttgaggttacagtgatctcacgctcactgatgatcatgccactgcactccaaacttaagtgacaacccatgtttttaaaaaaaaaaaaaagtcaccgcgagttcgattcaaacagtgtgaaggaggaagcaactaattatctccctctcctgatttttcataattttattaaatcatcactgggaaaactaatggtttgcgtatcacacaattacactacaatctgataggagtggtaaaaccagccaatggaatccaggtaaagtacaaaaacgccaccttttattgtcctgtcttatttctcgggaaggagggttctactttacacatttcatgagccagcagtggacttgagttacaatgtgtaggttccttgtggttatagctgcagaagaagccatcaaattcttgaggacttgacatctctcggaaagaagcaaactagtagactgatgagctggattgcttagattgataacatttacaaataggagtccagttgacatgctattaatgttgaaataaccatgcctgtactggtcagtgagttcggtcagctggttggaataccagttccagagctttaggcgacacatttgaattgagttatcattgtagagagtcatggctccatcagctatggttatcttctttggtctgaatgcctatcagtccttaccagctgtagcagccactgcttggtaaaactttgccacgaagtctggctcactgaactccagctgtctgacaaattcattgcgctcctgctcagcccagcctcgaaaccactgatcccaaagatgtagctggcactcaaagatagaaggtggtcggtctgccccagacacactaagctgctccagactatccagcagtggttgtaatttttctggcactgccttagctaccaggtcctctaggaaacgttcacgctggggacctgaccaattggcaaaccagtgaagaatacacttcatctcctgggaggtgatgtaagacatcagaggaggggaagggttagtattgtgtggtactgagggtaagagagatgggaaggatagtggcattgaagaggatgactccagtggcatcctccccttttctctcgaagggcacccgaagattgtcacgagtccttagactccaactactgcggcagcttccaaatttcctgaaaaccctaagctgggccagcccggcagcccac

SEQ ID NO: 11011 - RNA, 1175 nt, Homo sapiens
  source 1..1175: mol_type = other RNA
ctgaatagctgggactacaggtgcacaccaccatgcctggctaagttttgtattttttgtagagatggggttccgccatgttgcccaggctggtctcaaactcctgggctcaagtgatccactcacctcggccttccaaagcgctgggattacaggcgtgagccaccatgcccaaccaagattatttttaaaaattagaacatactcaccagggttgtagacatagatgggttgaaaatattctaggttctcaatacagttttcggtttttagtccacctagaaatgcacactcataatggctgcaggtcttgtttatgctttgaaggataaggttattgccagccccctcctgtgacacttgaaaaacctcattcagaggtattaaagtaattctttcactttctttatcaagaaaattttcaatgtcaactccaaggcatgtgtagatggataacacagtgagctggtcattagcagcctgaggtttggctgaatatgccaaggtaaaatggccaaacctggcttggtttagccctccaaatgtaaatgaagtgccctggcttgttctatataccacagttttggaactggcctcacaaggttttctcagcaactgcagggctcttgtgaggtaaaagtggaaagctttgaactggaagccatagatataatcttctcgagattggccagccatcttcacagcttcactgaacagatggtaaaagggagtttgctcttgagcttcggaaatatatgccatcagggctattccatggttatccttaaaattcatagggagaaagatttgagtctttcgggctgcccatttggcttttgcattttcccacacagtatctaattgctggtggcttgctttttcctcctttagcagttggggaacgtatttaatttccatcctgtccgtacatttcaggtattcatcatcaaatgcattatctgccatgtctaacacttcagccttcacctggaaaatgtccactagaatcatggttgccagcagcatggtgactatttcaaaatgtcccgtcttcatttttctcttctggcttttgtgcctttggaggaagtttaagtgatgctaggcctcaaactgactccccactctcagttgtggtaagcaagtcttcaggatgggatgttgttgacagtgag

SEQ ID NO: 11012 - RNA, 824 nt, Homo sapiens
  source 1..824: mol_type = other RNA
ctgaatagctgggactacaggtgcacaccaccatgcctggctaatttttgtatttttagttgagatggggtttcaccatgttggtcaggctggtatcgaactcctggcctcaagtgatccacctgcctcagcctcccaaagtgctgggattagaggtgtaagccactgcgcccggccttattgagtgttaactatgtgccagcggcacaaattatctcagttgttttttttgtcacaaccttttgaagggggtgggcctcatacaagatgagaaaaccatgactcaggcgatgcaggccttacgcggaagccctgtgccatccgctgccttctgactgacggtgttgctccacctgtagtcctagctaccgaggaggctgaggtgggaggatcgcttgagcctgggaggccaaggctgcagtgagctgtgatcatgccactgcagtccagcctgggcaacagagtgagatcctggatcagtgttgccttccagagagggagggagagacagctgggagataaactcacagtggcccagacccacatgacccagtggatgggcaccgtgaggaggtccttccaggaagccctcaatttggtgaccaccacggtgggccacgaacggacgagtgcagagtcggccagccggacccccttcaagcgtacttcctccttccgacacctggcttcccggagtcgggaatccttccgccgcttctctgctcgcagccaacagagattttcttcactgggaaagaggcacgtagcaataattcctctctcctgaagtcagtcaggacatttttgctggagtcgacgtctgt

SEQ ID NO: 11013 - RNA, 5027 nt, Homo sapiens
  source 1..5027: mol_type = other RNA
ctgaatagctgggactacaggtgcacaccaccattcctggctaatttttttatttttatttttgtagagatggaatcccattatgttacccaggctggtcttgaacttctgggctcaagccatcctcccaccttggcctcctgaagtgctgggattataggcgtgagccacggcacctggccaacaagtatttactgaatgtccactggctttctgagatctaggatttggtctaaaagatatctcgaggctctttcccaatctattgctctaagaaatgttttacagtaaactaggatggtaacctaaaaaagaaaaatatatgacaacctaaaaaaaacttaacaacacaaaatgactgaaaagaactcaggtaaaaggagaaaaacatacagaacttaaaatataaattaacttctttcaaaataaaaatagtttaatttccatcaagtatagcgatatgcagtctataaattctcacaaacacagctttaaaaagtgcaagttgcaggaactatgataaatttgaaaataacaatctttttattagacatctgaccaagaggatgctgtaagatgcgcaatgtcaggttatatggagcttattcacatgcttcttgctatactaaatatacactaaatggcttttatttaaaatttcataaaaggaacatttcattaaaaccaatttaaattctacaactactaagaacaaataaaactagtagaggtgaacaaatctctcttctccagtcgactggacagcaggattactgagtagtaggtaggccgagtcttcttcacccccttattatttggtgaggaagtcaactgtgagaagtgactcgaactgtcagaagaaatgagaaaagtgcttgggtctatgggcagggtactaagatctacagcgcctgttgccttagtttaatctggatcctctgaagagctatctatctcaaggccagcattttcttcctgccaacttagattactgtgacgaggggcaccttcatccaggccaagcgtgttcagctcttcgaagctgaagttgagtgtgtagggcgtctggctggagagctcggtgtgaggcagctcgttgtgggaagcgcggcgagcaggctcaccgtgcggggctgggccactgctgctctcactgaggaaacgtgggtcttcagggaccacgtggctttctgcgtttctcatttctagtactgtgcttctgaaaaggtgccagtctccaaaattcatattcatctctttcttcagctcatcaatgttacactgagctaacacacggccatttatgtttgcctttttgatcgtggtacaatactgaggcagcatactctggtccagcccttctatttgtttcagcttctcacatactgcatccacattcagtgaattcagtaataccactgggcctggggctgggcctgaccccctgttgtagaagggatgctgagggcccgtcatgccgctgtaatagctgctgtgaggctgtggtgacaccactccacctgcgaagggcccattgaaggacgtggaagagcacacggatgggggctggctgtaccctgatggcgccctaggaggaccctcatgtagagggagcggggggtacgccagtcctccaatactgatctgctctctggcagcacgaacatctgcaataatttcccgtagtttgggatctaggtttacagtgcatggcaaaaagacttttacatctcgagccacaagaactggggtccttgaagacaaaaacacttcaaaatttcttatatctccatcaatttcaagaagtggctcaacatccttagttgttggaatattctttgatattctttcgtagatggtttttaatgtcatttgatctggaataccttcagtctcttccaaatataatatgagccatgaagtccggtatggccactgctcagtaaggttgatccagctagcaagcctgtcccagttgaaactaatctgattggctctcagtaatcgtcctgtcacagaaacaatattaagtaatcttctcatggtctggggactgatgtcactgaaccagtcctcggtaaccagcagttttgtaagatcaaaggacatctggcgagtgatggtcctctgcatctgccttcttcggtaagtgtcccgtctattgagggctgtcttgctaccaagttttgtcatctccccaaggctgttctgtgaaactcttctgtcagcatcttcctgtatccctgtagtatctgagcatggaacgtctccatttgttgctgaagttacgagaaattttcttgcattgcttagtccacgactattaaggaacacaggcaagtggactatgttgcgcatgtagtcatggccatttatatttgaatcccgaagcacactattgaggttctggttaattgcctttatgataatatgtggatcacttgcaaaaatggcaatgaacgggccttttgaaaacagaactcggacagtgtccagcatctgaaggactttgtcctgctcacaggcatctaatccatcgatgatgaccaccagccttgtctgattctgagtgaagctgtcaatggtttttgccatcctggccatcaattccacttcacatttaagaactttcatgaatccttcacttttcaatttgtgcagtttggaggctgcattatggaggcgttttctttgggaattcaggagcgagtccagcacttgccaccatgtacgacagttcaacacaaaggccaatcccactacagatgcgattgatatgaggacagcatttacagtcagatgctttgggtcaactctaaatatagccagaagagtaattccagatataatgcagccaatgataaaaaggaagatgacaaaagatgggagacaacatgtttttttccatttctttttaccctgagtatcttcagtcttgaatactcgaaaaagcctggttgccaaaaagccaaactctctttcacaagcatccgagagggttgcaatcatttcagccagagaagtttctccacctacactggacagtctattgtaatctgtaaacaaaaacctcacaggtaaagctttagtagtctgctctggcaactcaggtggattcacaaacatcaatttaaggaggagttccaaatatccaatatgtcttgccaatctagtgctgaggacccaggcccaattccaactctctccttctcttcgtccaccaaagtaaatgacaataaagaatatatataagagagccaagaagctcagtgacactgctattccaagatttgggtggaccgtgaaggcaaacaataaaccaagccctccacaaagtagcagggtaagaaacactatgagccatgagaactgaaagagaggctcaatctgttgtccggcgaaggttttcatttcgtcttctagtttcttgagtaagaaagatttcccacttccccactgtgcatataaccccacacaaatgggtggctgcatggtaggctcactgagaatatctgccagggcactgctatataaatcatatccaagcatgtcaccgtctgtttcagtaggagacaagtgtctggctccaaatatttgagttaaaatactcttctgatggctacagtcaatattataaggagtctcgcctgctttgttgggcctataaagtaatcgcccatctttgggatttcttaaaagcagttctgccagtttccggctccttccacgaatagcaatatgcaagggagtatctcctttcttatctacagcagacactttagcacctttatctagcagcagctccaccacttcaatgtttctcatcttggtagcctttataagtggcgtttcaccatcctttgtgcatatttcagtgtcaggattgcactgtaagatatctctcaccattgttgcatttcctttctcaacagcccaatacaaagcagttttattatcctgtcctctaatgtctatatcagcatatttttggagaagcgctcgaacaatttcaacatgaccacctctgacagcgccaatcaacacagtatccccactcctgtcaggtatgttcacatatgttccagcgtcgagcagatcctgcacaatctccgtatgtccctcctttgatgcaatcatcaaagctgtatttccatctttatctgttaagtttacatttggattcctcttcaaaatttcttttactgactgtgtgtaacctcctttcactgccacaataagtgcagtcattgaattagctccttcttgatccacatcagctcccatggccaataaatgtttcacacattccaaatgaccctttcgtgcagcccaaactaaaggggtggttccatacttatcagagcagttgactttagcaccattttgcagtaaaagatgaactatatctgcatggcctctccctgctgcccaaatgattgggtaaacactgtacagaccagtgacacttggattggcaccatgagaaagaagcaactctactacgtcagtacggcctttgtaacatgcccacataagagctgtccatcctcccatatcacggtgctccaagttaaccccacatttcagtagttcctctacgatgtgcacatgcccttctttcgatgcagatataagtgctgtccaattatccaaatcttccagattgcagttagctccattcttaattaattccttcactatttccagattgccttgttcggcagctatcatcagtggagtctggccacactcatttctctcatctacatctttgcatttttcaagaagagctttcagagcaggaatgttttcttcctctacataatttatgacgctctgtgatatcaaaactgacattttcacagaaagctgcaattaactttatttgaatacctggtcctcagctccggcggaacgggcccgctcggctgcaggcgatgtcagaggacggggaagcaagagacggcgactgcaagcgcgtcgccctcaccacacccggcggccatattcttccctctccgcgaact

SEQ ID NO: 11014 - RNA, 5212 nt, Homo sapiens
  source 1..5212: mol_type = other RNA
ctgaatagctgggactacaggtgcacaccaccattcctggctaatttttttatttttatttttgtagagatggaatcccattatgttacccaggctggtcttgaacttctgggctcaagccatcctcccaccttggcctcctgaagtgctgggattataggcgtgagccacggcacctggccaacaagtatttactgaatgtccactggctttctgagatctaggatttggtctaaaagatatctcgaggctctttcccaatctattgctctaagaaatgttttacagtaaactaggatggtaacctaaaaaagaaaaatatatgacaacctaaaaaaaacttaacaacacaaaatgactgaaaagaactcaggtaaaaggagaaaaacatacagaacttaaaatataaattaacttctttcaaaataaaaatagtttaatttccatcaagtatagcgatatgcagtctataaattctcacaaacacagctttaaaaagtgcaagttgcaggaactatgataaatttgaaaataacaatctttttattagacatctgaccaagaggatgctgtaagatgcgcaatgtcaggttatatggagcttattcacatgcttcttgctatactaaatatacactaaatggcttttatttaaaatttcataaaaggaacatttcattaaaaccaatttaaattctacaactactaagaacaaataaaactagtagaggtgaacaaatctctcttctccagtcgactggacagcaggattactgagtagtaggtaggccgagtcttcttcacccccttattatttggtgaggaagtcaactgtgagaagtgactcgaacttagtttaatctggatcctctgaagagctatctatctcaaggccagcattttcttcctgagtctgctcatgctgcccccgcaaaagaacagtatccccactggtttcttcccttccgcccagtgtcggcgtgcgcctgccaacttagattactgtgacgaggggcaccttcatccaggccaagcgtgttcagctcttcgaagctgaagttgagtgtgtagggcgtctggctggagagctcggtgtgaggcagctcgttgtgggaagcgcggcgagcaggctcaccgtgcggggctgggccactgctgctctcactgaggaaacgtgggtcttcagggaccacgtggctttctgcgtttctcatttctagtactgtgcttctgaaaaggtgccagtctccaaaattcatattcatctctttcttcagctcatcaatgttacactgagctaacacacggccatttatgtttgcctttttgatcgtggtacaatactgaggcagcatactctggtccagcccttctatttgtttcagcttctcacatactgcatccacattcagtgaattcagtaataccactgggcctggggctgggcctgaccccctcgaggagtctgtgggtgaagaaagcccctcagcagcatcctccttgataacttctaggccattgttctgatctctgggcaaactcgtttttactgatggacgtgagatgagatgttgggagccgccagggtaataccttggcgtgtaaaggtatggggcaaagaatggcctgttgtagaagggatgctgagggcccgtcatgccgctgtaatagctgctgtgaggctgtggtgacaccactccacctgcgaagggcccattgaaggacgtggaagagcacacggatgggggctggctgtaccctgatggcgccctaggaggaccctcatgtagagggagcggggggtacgccagtcctccaatactgatctgctctctggcagcacgaacatctgcaataatttcccgtagtttgggatctaggtttacagtgcatggcaaaaagacttttacatctcgagccacaagaactggggtccttgaagacaaaaacacttcaaaatttcttatatctccatcaatttcaagaagtggctcaacatccttagttgttggaatattctttgatattctttcgtagatggtttttaatgtcatttgatctggaataccttcagtctcttccaaatataatatgagccatgaagtccggtatggccactgctcagtaaggttgatccagctagcaagcctgtcccagttgaaactaatctgattggctctcagtaatcgtcctgtcacagaaacaatattaagtaatcttctcatggtctggggactgatgtcactgaaccagtcctcggtaaccagcagttttgtaagatcaaaggacatctggcgagtgatggtcctctgcatctgccttcttcggtaagtgtcccgtctattgagggctgtcttgctaccaagttttgtcatctccccaaggctgttctgtgaaactcttctgtcagcatcttcctgtatccctgtagtatctgagcatggaacgtctccatttgttgctgaagttacgagaaattttcttgcattgcttagtccacgactattaaggaacacaggcaagtggactatgttgcgcatgtagtcatggccatttatatttgaatcccgaagcacactattgaggttctggttaattgcctttatgataatatgtggatcacttgcaaaaatggcaatgaacgggccttttgaaaacagaactcggacagtgtccagcatctgaaggactttgtcctgctcacaggcatctaatccatcgatgatgaccaccagccttgtctgattctgagtgaagctgtcaatggtttttgccatcctggccatcaattccacttcacatttaagaactttcatgaatccttcacttttcaatttgtgcagtttggaggctgcattatggaggcgttttctttgggaattcaggagcgagtccagcacttgccaccatgtacgacagttcaacacaaaggccaatcccactacagatgcgattgatatgaggacagcatttacagtcagatgctttgggtcaactctaaatatagccagaagagtaattccagatataatgcagccaatgataaaaaggaagatgacaaaagatgggagacaacatgtttttttccatttctttttaccctgagtatcttcagtcttgaatactcgaaaaagcctggttgccaaaaagccaaactctctttcacaagcatccgagagggttgcaatcatttcagccagagaagtttctccacctacactggacagtctattgtaatctgtaaacaaaaacctcacaggtaaagctttagtagtctgctctggcaactcaggtggattcacaaacatcaatttaaggaggagttccaaatatccaatatgtcttgccaatctagtgctgaggacccaggcccaattccaactctctccttctcttcgtccaccaaagtaaatgacaataaagaatatatataagagagccaagaagctcagtgacactgctattccaagatttgggtggaccgtgaaggcaaacaataaaccaagccctccacaaagtagcagggtaagaaacactatgagccatgagaactgaaagagaggctcaatctgttgtccggcgaaggttttcatttcgtcttctagtttcttgagtaagaaagatttcccacttccccactgtgcatataaccccacacaaatgggtggctgcatggtaggctcactgagaatatctgccagggcactgctatataaatcatatccaagcatgtcaccgtctgtttcagtaggagacaagtgtctggctccaaatatttgagttaaaatactcttctgatggctacagtcaatattataaggagtctcgcctgctttgttgggcctataaagtaatcgcccatctttgggatttcttaaaagcagttctgccagtttccggctccttccacgaatagcaatatgcaagggagtatctcctttcttatctacagcagacactttagcacctttatctagcagcagctccaccacttcaatgtttctcatcttggtagcctttataagtggcgtttcaccatcctttgtgcatatttcagtgtcaggattgcactgtaagatatctctcaccattgttgcatttcctttctcaacagcccaatacaaagcagttttattatcctgtcctctaatgtctatatcagcatatttttggagaagcgctcgaacaatttcaacatgaccacctctgacagcgccaatcaacacagtatccccactcctgtcaggtatgttcacatatgttccagcgtcgagcagatcctgcacaatctccgtatgtccctcctttgatgcaatcatcaaagctgtatttccatctttatctgttaagtttacatttggattcctcttcaaaatttcttttactgactgtgtgtaacctcctttcactgccacaataagtgcagtcattgaattagctccttcttgatccacatcagctcccatggccaataaatgtttcacacattccaaatgaccctttcgtgcagcccaaactaaaggggtggttccatacttatcagagcagttgactttagcaccattttgcagtaaaagatgaactatatctgcatggcctctccctgctgcccaaatgattgggtaaacactgtactgcagaccagtgacacttggattggcaccatgagaaagaagcaactctactacgtcagtacggcctttgtaacatgcccacataagagctgtccatcctcccatatcacggtgctccaagttaaccccacatttcagtagttcctctacgatgtgcacatgcccttctttcgatgcagatataagtgctgtccaattatccaaatcttccagattgcagttagctccattcttaattaattccttcactatttccagattgccttgttcggcagctatcatcagtggagtctggccacactcatttctctcatctacatctttgcatttttcaagaagagctttcagagcaggaatgttttcttcctctacataatttatgacgctctgtgatatcaaaactgacattttcacagaaagctgcaattaactttatttgaatacctggtcctcagctccggcggaacgggcccgctcggctgcaggcgatgtcagaggacggggaagcaagagacggcgactgcaagcgcgtcgccctcaccacacccggcggccatattcttccctctccgcgaact

SEQ ID NO: 11015 - RNA, 5038 nt, Homo sapiens
  source 1..5038: mol_type = other RNA
ctgaatagctgggactacaggtgcacaccaccattcctggctaatttttttatttttatttttgtagagatggaatcccattatgttacccaggctggtcttgaacttctgggctcaagccatcctcccaccttggcctcctgaagtgctgggattataggcgtgagccacggcacctggccaacaagtatttactgaatgtccactggctttctgagatctaggatttggtctaaaagatatctcgaggctctttcccaatctattgctctaagaaatgttttacagtaaactaggatggtaacctaaaaaagaaaaatatatgacaacctaaaaaaaacttaacaacacaaaatgactgaaaagaactcaggtaaaaggagaaaaacatacagaacttaaaatataaattaacttctttcaaaataaaaatagtttaatttccatcaagtatagcgatatgcagtctataaattctcacaaacacagctttaaaaagtgcaagttgcaggaactatgataaatttgaaaataacaatctttttattagacatctgaccaagaggatgctgtaagatgcgcaatgtcaggttatatggagcttattcacatgcttcttgctatactaaatatacactaaatggcttttatttaaaatttcataaaaggaacatttcattaaaaccaatttaaattctacaactactaagaacaaataaaactagtagaggtgaacaaatctctcttctccagtcgactggacagcaggattactgagtagtaggtaggccgagtcttcttcacccccttattatttggtgaggaagtcaactgtgagaagtgactcgaacttagtttaatctggatcctctgaagagctatctatctcaaggccagcattttcttcctgagtctgctcatgctgcccccgcaaaagaacagtatccccactggtttcttcccttccgcccagtgtcggcgtgcgcctgccaacttagattactgtgacgaggggcaccttcatccaggccaagcgtgttcagctcttcgaagctgaagttgagtgtgtagggcgtctggctggagagctcggtgtgaggcagctcgttgtgggaagcgcggcgagcaggctcaccgtgcggggctgggccactgctgctctcactgaggaaacgtgggtcttcagggaccacgtggctttctgcgtttctcatttctagtactgtgcttctgaaaaggtgccagtctccaaaattcatattcatctctttcttcagctcatcaatgttacactgagctaacacacggccatttatgtttgcctttttgatcgtggtacaatactgaggcagcatactctggtccagcccttctatttgtttcagcttctcacatactgcatccacattcagtgaattcagtaataccactgggcctggggctgggcctgaccccctgttgtagaagggatgctgagggcccgtcatgccgctgtaatagctgctgtgaggctgtggtgacaccactccacctgcgaagggcccattgaaggacgtggaagagcacacggatgggggctggctgtaccctgatggcgccctaggaggaccctcatgtagagggagcggggggtacgccagtcctccaatactgatctgctctctggcagcacgaacatctgcaataatttcccgtagtttgggatctaggtttacagtgcatggcaaaaagacttttacatctcgagccacaagaactggggtccttgaagacaaaaacacttcaaaatttcttatatctccatcaatttcaagaagtggctcaacatccttagttgttggaatattctttgatattctttcgtagatggtttttaatgtcatttgatctggaataccttcagtctcttccaaatataatatgagccatgaagtccggtatggccactgctcagtaaggttgatccagctagcaagcctgtcccagttgaaactaatctgattggctctcagtaatcgtcctgtcacagaaacaatattaagtaatcttctcatggtctggggactgatgtcactgaaccagtcctcggtaaccagcagttttgtaagatcaaaggacatctggcgagtgatggtcctctgcatctgccttcttcggtaagtgtcccgtctattgagggctgtcttgctaccaagttttgtcatctccccaaggctgttctgtgaaactcttctgtcagcatcttcctgtatccctgtagtatctgagcatggaacgtctccatttgttgctgaagttacgagaaattttcttgcattgcttagtccacgactattaaggaacacaggcaagtggactatgttgcgcatgtagtcatggccatttatatttgaatcccgaagcacactattgaggttctggttaattgcctttatgataatatgtggatcacttgcaaaaatggcaatgaacgggccttttgaaaacagaactcggacagtgtccagcatctgaaggactttgtcctgctcacaggcatctaatccatcgatgatgaccaccagccttgtctgattctgagtgaagctgtcaatggtttttgccatcctggccatcaattccacttcacatttaagaactttcatgaatccttcacttttcaatttgtgcagtttggaggctgcattatggaggcgttttctttgggaattcaggagcgagtccagcacttgccaccatgtacgacagttcaacacaaaggccaatcccactacagatgcgattgatatgaggacagcatttacagtcagatgctttgggtcaactctaaatatagccagaagagtaattccagatataatgcagccaatgataaaaaggaagatgacaaaagatgggagacaacatgtttttttccatttctttttaccctgagtatcttcagtcttgaatactcgaaaaagcctggttgccaaaaagccaaactctctttcacaagcatccgagagggttgcaatcatttcagccagagaagtttctccacctacactggacagtctattgtaatctgtaaacaaaaacctcacaggtaaagctttagtagtctgctctggcaactcaggtggattcacaaacatcaatttaaggaggagttccaaatatccaatatgtcttgccaatctagtgctgaggacccaggcccaattccaactctctccttctcttcgtccaccaaagtaaatgacaataaagaatatatataagagagccaagaagctcagtgacactgctattccaagatttgggtggaccgtgaaggcaaacaataaaccaagccctccacaaagtagcagggtaagaaacactatgagccatgagaactgaaagagaggctcaatctgttgtccggcgaaggttttcatttcgtcttctagtttcttgagtaagaaagatttcccacttccccactgtgcatataaccccacacaaatgggtggctgcatggtaggctcactgagaatatctgccagggcactgctatataaatcatatccaagcatgtcaccgtctgtttcagtaggagacaagtgtctggctccaaatatttgagttaaaatactcttctgatggctacagtcaatattataaggagtctcgcctgctttgttgggcctataaagtaatcgcccatctttgggatttcttaaaagcagttctgccagtttccggctccttccacgaatagcaatatgcaagggagtatctcctttcttatctacagcagacactttagcacctttatctagcagcagctccaccacttcaatgtttctcatcttggtagcctttataagtggcgtttcaccatcctttgtgcatatttcagtgtcaggattgcactgtaagatatctctcaccattgttgcatttcctttctcaacagcccaatacaaagcagttttattatcctgtcctctaatgtctatatcagcatatttttggagaagcgctcgaacaatttcaacatgaccacctctgacagcgccaatcaacacagtatccccactcctgtcaggtatgttcacatatgttccagcgtcgagcagatcctgcacaatctccgtatgtccctcctttgatgcaatcatcaaagctgtatttccatctttatctgttaagtttacatttggattcctcttcaaaatttcttttactgactgtgtgtaacctcctttcactgccacaataagtgcagtcattgaattagctccttcttgatccacatcagctcccatggccaataaatgtttcacacattccaaatgaccctttcgtgcagcccaaactaaaggggtggttccatacttatcagagcagttgactttagcaccattttgcagtaaaagatgaactatatctgcatggcctctccctgctgcccaaatgattgggtaaacactgtacagaccagtgacacttggattggcaccatgagaaagaagcaactctactacgtcagtacggcctttgtaacatgcccacataagagctgtccatcctcccatatcacggtgctccaagttaaccccacatttcagtagttcctctacgatgtgcacatgcccttctttcgatgcagatataagtgctgtccaattatccaaatcttccagattgcagttagctccattcttaattaattccttcactatttccagattgccttgttcggcagctatcatcagtggagtctggccacactcatttctctcatctacatctttgcatttttcaagaagagctttcagagcaggaatgttttcttcctctacataatttatgacgctctgtgatatcaaaactgacattttcacagaaagctgcaattaactttatttgaatacctggtcctcagctccggcggaacgggcccgctcggctgcaggcgatgtcagaggacggggaagcaagagacggcgactgcaagcgcgtcgccctcaccacacccggcggccatattcttccctctccgcgaact

SEQ ID NO: 11016 - RNA, 4959 nt, Homo sapiens
  source 1..4959: mol_type = other RNA
ctgaatagctgggactacaggtgcacaccaccattcctggctaatttttttatttttatttttgtagagatggaatcccattatgttacccaggctggtcttgaacttctgggctcaagccatcctcccaccttggcctcctgaagtgctgggattataggcgtgagccacggcacctggccaacaagtatttactgaatgtccactggctttctgagatctaggatttggtctaaaagatatctcgaggctctttcccaatctattgctctaagaaatgttttacagtaaactaggatggtaacctaaaaaagaaaaatatatgacaacctaaaaaaaacttaacaacacaaaatgactgaaaagaactcaggtaaaaggagaaaaacatacagaacttaaaatataaattaacttctttcaaaataaaaatagtttaatttccatcaagtatagcgatatgcagtctataaattctcacaaacacagctttaaaaagtgcaagttgcaggaactatgataaatttgaaaataacaatctttttattagacatctgaccaagaggatgctgtaagatgcgcaatgtcaggttatatggagcttattcacatgcttcttgctatactaaatatacactaaatggcttttatttaaaatttcataaaaggaacatttcattaaaaccaatttaaattctacaactactaagaacaaataaaactagtagaggtgaacaaatctctcttctccagtcgactggacagcaggattactgagtagtaggtaggccgagtcttcttcacccccttattatttggtgaggaagtcaactgtgagaagtgactcgaacttagtttaatctggatcctctgaagagctatctatctcaaggccagcattttcttcctgccaacttagattactgtgacgaggggcaccttcatccaggccaagcgtgttcagctcttcgaagctgaagttgagtgtgtagggcgtctggctggagagctcggtgtgaggcagctcgttgtgggaagcgcggcgagcaggctcaccgtgcggggctgggccactgctgctctcactgaggaaacgtgggtcttcagggaccacgtggctttctgcgtttctcatttctagtactgtgcttctgaaaaggtgccagtctccaaaattcatattcatctctttcttcagctcatcaatgttacactgagctaacacacggccatttatgtttgcctttttgatcgtggtacaatactgaggcagcatactctggtccagcccttctatttgtttcagcttctcacatactgcatccacattcagtgaattcagtaataccactgggcctggggctgggcctgaccccctgttgtagaagggatgctgagggcccgtcatgccgctgtaatagctgctgtgaggctgtggtgacaccactccacctgcgaagggcccattgaaggacgtggaagagcacacggatgggggctggctgtaccctgatggcgccctaggaggaccctcatgtagagggagcggggggtacgccagtcctccaatactgatctgctctctggcagcacgaacatctgcaataatttcccgtagtttgggatctaggtttacagtgcatggcaaaaagacttttacatctcgagccacaagaactggggtccttgaagacaaaaacacttcaaaatttcttatatctccatcaatttcaagaagtggctcaacatccttagttgttggaatattctttgatattctttcgtagatggtttttaatgtcatttgatctggaataccttcagtctcttccaaatataatatgagccatgaagtccggtatggccactgctcagtaaggttgatccagctagcaagcctgtcccagttgaaactaatctgattggctctcagtaatcgtcctgtcacagaaacaatattaagtaatcttctcatggtctggggactgatgtcactgaaccagtcctcggtaaccagcagttttgtaagatcaaaggacatctggcgagtgatggtcctctgcatctgccttcttcggtaagtgtcccgtctattgagggctgtcttgctaccaagttttgtcatctccccaaggctgttctgtgaaactcttctgtcagcatcttcctgtatccctgtagtatctgagcatggaacgtctccatttgttgctgaagttacgagaaattttcttgcattgcttagtccacgactattaaggaacacaggcaagtggactatgttgcgcatgtagtcatggccatttatatttgaatcccgaagcacactattgaggttctggttaattgcctttatgataatatgtggatcacttgcaaaaatggcaatgaacgggccttttgaaaacagaactcggacagtgtccagcatctgaaggactttgtcctgctcacaggcatctaatccatcgatgatgaccaccagccttgtctgattctgagtgaagctgtcaatggtttttgccatcctggccatcaattccacttcacatttaagaactttcatgaatccttcacttttcaatttgtgcagtttggaggctgcattatggaggcgttttctttgggaattcaggagcgagtccagcacttgccaccatgtacgacagttcaacacaaaggccaatcccactacagatgcgattgatatgaggacagcatttacagtcagatgctttgggtcaactctaaatatagccagaagagtaattccagatataatgcagccaatgataaaaaggaagatgacaaaagatgggagacaacatgtttttttccatttctttttaccctgagtatcttcagtcttgaatactcgaaaaagcctggttgccaaaaagccaaactctctttcacaagcatccgagagggttgcaatcatttcagccagagaagtttctccacctacactggacagtctattgtaatctgtaaacaaaaacctcacaggtaaagctttagtagtctgctctggcaactcaggtggattcacaaacatcaatttaaggaggagttccaaatatccaatatgtcttgccaatctagtgctgaggacccaggcccaattccaactctctccttctcttcgtccaccaaagtaaatgacaataaagaatatatataagagagccaagaagctcagtgacactgctattccaagatttgggtggaccgtgaaggcaaacaataaaccaagccctccacaaagtagcagggtaagaaacactatgagccatgagaactgaaagagaggctcaatctgttgtccggcgaaggttttcatttcgtcttctagtttcttgagtaagaaagatttcccacttccccactgtgcatataaccccacacaaatgggtggctgcatggtaggctcactgagaatatctgccagggcactgctatataaatcatatccaagcatgtcaccgtctgtttcagtaggagacaagtgtctggctccaaatatttgagttaaaatactcttctgatggctacagtcaatattataaggagtctcgcctgctttgttgggcctataaagtaatcgcccatctttgggatttcttaaaagcagttctgccagtttccggctccttccacgaatagcaatatgcaagggagtatctcctttcttatctacagcagacactttagcacctttatctagcagcagctccaccacttcaatgtttctcatcttggtagcctttataagtggcgtttcaccatcctttgtgcatatttcagtgtcaggattgcactgtaagatatctctcaccattgttgcatttcctttctcaacagcccaatacaaagcagttttattatcctgtcctctaatgtctatatcagcatatttttggagaagcgctcgaacaatttcaacatgaccacctctgacagcgccaatcaacacagtatccccactcctgtcaggtatgttcacatatgttccagcgtcgagcagatcctgcacaatctccgtatgtccctcctttgatgcaatcatcaaagctgtatttccatctttatctgttaagtttacatttggattcctcttcaaaatttcttttactgactgtgtgtaacctcctttcactgccacaataagtgcagtcattgaattagctccttcttgatccacatcagctcccatggccaataaatgtttcacacattccaaatgaccctttcgtgcagcccaaactaaaggggtggttccatacttatcagagcagttgactttagcaccattttgcagtaaaagatgaactatatctgcatggcctctccctgctgcccaaatgattgggtaaacactgtacagaccagtgacacttggattggcaccatgagaaagaagcaactctactacgtcagtacggcctttgtaacatgcccacataagagctgtccatcctcccatatcacggtgctccaagttaaccccacatttcagtagttcctctacgatgtgcacatgcccttctttcgatgcagatataagtgctgtccaattatccaaatcttccagattgcagttagctccattcttaattaattccttcactatttccagattgccttgttcggcagctatcatcagtggagtctggccacactcatttctctcatctacatctttgcatttttcaagaagagctttcagagcaggaatgttttcttcctctacataatttatgacgctctgtgatatcaaaactgacattttcacagaaagctgcaattaactttatttgaatacctggtcctcagctccggcggaacgggcccgctcggctgcaggcgatgtcagaggacggggaagcaagagacggcgactgcaagcgcgtcgccctcaccacacccggcggccatattcttccctctccgcgaact

SEQ ID NO: 11017 - RNA, 4962 nt, Homo sapiens
  source 1..4962: mol_type = other RNA
ctgaatagctgggactacaggtgcacaccaccattcctggctaatttttttatttttatttttgtagagatggaatcccattatgttacccaggctggtcttgaacttctgggctcaagccatcctcccaccttggcctcctgaagtgctgggattataggcgtgagccacggcacctggccaacaagtatttactgaatgtccactggctttctgagatctaggatttggtctaaaagatatctcgaggctctttcccaatctattgctctaagaaatgttttacagtaaactaggatggtaacctaaaaaagaaaaatatatgacaacctaaaaaaaacttaacaacacaaaatgactgaaaagaactcaggtaaaaggagaaaaacatacagaacttaaaatataaattaacttctttcaaaataaaaatagtttaatttccatcaagtatagcgatatgcagtctataaattctcacaaacacagctttaaaaagtgcaagttgcaggaactatgataaatttgaaaataacaatctttttattagacatctgaccaagaggatgctgtaagatgcgcaatgtcaggttatatggagcttattcacatgcttcttgctatactaaatatacactaaatggcttttatttaaaatttcataaaaggaacatttcattaaaaccaatttaaattctacaactactaagaacaaataaaactagtagaggtgaacaaatctctcttctccagtcgactggacagcaggattactgagtagtaggtaggccgagtcttcttcacccccttattatttggtgaggaagtcaactgtgagaagtgactcgaacttagtttaatctggatcctctgaagagctatctatctcaaggccagcattttcttcctgccaacttagattactgtgacgaggggcaccttcatccaggccaagcgtgttcagctcttcgaagctgaagttgagtgtgtagggcgtctggctggagagctcggtgtgaggcagctcgttgtgggaagcgcggcgagcaggctcaccgtgcggggctgggccactgctgctctcactgaggaaacgtgggtcttcagggaccacgtggctttctgcgtttctcatttctagtactgtgcttctgaaaaggtgccagtctccaaaattcatattcatctctttcttcagctcatcaatgttacactgagctaacacacggccatttatgtttgcctttttgatcgtggtacaatactgaggcagcatactctggtccagcccttctatttgtttcagcttctcacatactgcatccacattcagtgaattcagtaataccactgggcctggggctgggcctgaccccctgttgtagaagggatgctgagggcccgtcatgccgctgtaatagctgctgtgaggctgtggtgacaccactccacctgcgaagggcccattgaaggacgtggaagagcacacggatgggggctggctgtaccctgatggcgccctaggaggaccctcatgtagagggagcggggggtacgccagtcctccaatactgatctgctctctggcagcacgaacatctgcaataatttcccgtagtttgggatctaggtttacagtgcatggcaaaaagacttttacatctcgagccacaagaactggggtccttgaagacaaaaacacttcaaaatttcttatatctccatcaatttcaagaagtggctcaacatccttagttgttggaatattctttgatattctttcgtagatggtttttaatgtcatttgatctggaataccttcagtctcttccaaatataatatgagccatgaagtccggtatggccactgctcagtaaggttgatccagctagcaagcctgtcccagttgaaactaatctgattggctctcagtaatcgtcctgtcacagaaacaatattaagtaatcttctcatggtctggggactgatgtcactgaaccagtcctcggtaaccagcagttttgtaagatcaaaggacatctggcgagtgatggtcctctgcatctgccttcttcggtaagtgtcccgtctattgagggctgtcttgctaccaagttttgtcatctccccaaggctgttctgtgaaactcttctgtcagcatcttcctgtatccctgtagtatctgagcatggaacgtctccatttgttgctgaagttacgagaaattttcttgcattgcttagtccacgactattaaggaacacaggcaagtggactatgttgcgcatgtagtcatggccatttatatttgaatcccgaagcacactattgaggttctggttaattgcctttatgataatatgtggatcacttgcaaaaatggcaatgaacgggccttttgaaaacagaactcggacagtgtccagcatctgaaggactttgtcctgctcacaggcatctaatccatcgatgatgaccaccagccttgtctgattctgagtgaagctgtcaatggtttttgccatcctggccatcaattccacttcacatttaagaactttcatgaatccttcacttttcaatttgtgcagtttggaggctgcattatggaggcgttttctttgggaattcaggagcgagtccagcacttgccaccatgtacgacagttcaacacaaaggccaatcccactacagatgcgattgatatgaggacagcatttacagtcagatgctttgggtcaactctaaatatagccagaagagtaattccagatataatgcagccaatgataaaaaggaagatgacaaaagatgggagacaacatgtttttttccatttctttttaccctgagtatcttcagtcttgaatactcgaaaaagcctggttgccaaaaagccaaactctctttcacaagcatccgagagggttgcaatcatttcagccagagaagtttctccacctacactggacagtctattgtaatctgtaaacaaaaacctcacaggtaaagctttagtagtctgctctggcaactcaggtggattcacaaacatcaatttaaggaggagttccaaatatccaatatgtcttgccaatctagtgctgaggacccaggcccaattccaactctctccttctcttcgtccaccaaagtaaatgacaataaagaatatatataagagagccaagaagctcagtgacactgctattccaagatttgggtggaccgtgaaggcaaacaataaaccaagccctccacaaagtagcagggtaagaaacactatgagccatgagaactgaaagagaggctcaatctgttgtccggcgaaggttttcatttcgtcttctagtttcttgagtaagaaagatttcccacttccccactgtgcatataaccccacacaaatgggtggctgcatggtaggctcactgagaatatctgccagggcactgctatataaatcatatccaagcatgtcaccgtctgtttcagtaggagacaagtgtctggctccaaatatttgagttaaaatactcttctgatggctacagtcaatattataaggagtctcgcctgctttgttgggcctataaagtaatcgcccatctttgggatttcttaaaagcagttctgccagtttccggctccttccacgaatagcaatatgcaagggagtatctcctttcttatctacagcagacactttagcacctttatctagcagcagctccaccacttcaatgtttctcatcttggtagcctttataagtggcgtttcaccatcctttgtgcatatttcagtgtcaggattgcactgtaagatatctctcaccattgttgcatttcctttctcaacagcccaatacaaagcagttttattatcctgtcctctaatgtctatatcagcatatttttggagaagcgctcgaacaatttcaacatgaccacctctgacagcgccaatcaacacagtatccccactcctgtcaggtatgttcacatatgttccagcgtcgagcagatcctgcacaatctccgtatgtccctcctttgatgcaatcatcaaagctgtatttccatctttatctgttaagtttacatttggattcctcttcaaaatttcttttactgactgtgtgtaacctcctttcactgccacaataagtgcagtcattgaattagctccttcttgatccacatcagctcccatggccaataaatgtttcacacattccaaatgaccctttcgtgcagcccaaactaaaggggtggttccatacttatcagagcagttgactttagcaccattttgcagtaaaagatgaactatatctgcatggcctctccctgctgcccaaatgattgggtaaacactgtactgcagaccagtgacacttggattggcaccatgagaaagaagcaactctactacgtcagtacggcctttgtaacatgcccacataagagctgtccatcctcccatatcacggtgctccaagttaaccccacatttcagtagttcctctacgatgtgcacatgcccttctttcgatgcagatataagtgctgtccaattatccaaatcttccagattgcagttagctccattcttaattaattccttcactatttccagattgccttgttcggcagctatcatcagtggagtctggccacactcatttctctcatctacatctttgcatttttcaagaagagctttcagagcaggaatgttttcttcctctacataatttatgacgctctgtgatatcaaaactgacattttcacagaaagctgcaattaactttatttgaatacctggtcctcagctccggcggaacgggcccgctcggctgcaggcgatgtcagaggacggggaagcaagagacggcgactgcaagcgcgtcgccctcaccacacccggcggccatattcttccctctccgcgaact

SEQ ID NO: 11018 - RNA, 5073 nt, Homo sapiens
  source 1..5073: mol_type = other RNA
ctgaatagctgggactacaggtgcacaccaccattcctggctaatttttttatttttatttttgtagagatggaatcccattatgttacccaggctggtcttgaacttctgggctcaagccatcctcccaccttggcctcctgaagtgctgggattataggcgtgagccacggcacctggccaacaagtatttactgaatgtccactggctttctgagatctaggatttggtctaaaagatatctcgaggctctttcccaatctattgctctaagaaatgttttacagtaaactaggatggtaacctaaaaaagaaaaatatatgacaacctaaaaaaaacttaacaacacaaaatgactgaaaagaactcaggtaaaaggagaaaaacatacagaacttaaaatataaattaacttctttcaaaataaaaatagtttaatttccatcaagtatagcgatatgcagtctataaattctcacaaacacagctttaaaaagtgcaagttgcaggaactatgataaatttgaaaataacaatctttttattagacatctgaccaagaggatgctgtaagatgcgcaatgtcaggttatatggagcttattcacatgcttcttgctatactaaatatacactaaatggcttttatttaaaatttcataaaaggaacatttcattaaaaccaatttaaattctacaactactaagaacaaataaaactagtagaggtgaacaaatctctcttctccagtcgactggacagcaggattactgagtagtaggtaggccgagtcttcttcacccccttattatttggtgaggaagtcaactgtgagaagtgactcgaacttagtttaatctggatcctctgaagagctatctatctcaaggccagcattttcttcctgccaacttagattactgtgacgaggggcaccttcatccaggccaagcgtgttcagctcttcgaagctgaagttgagtgtgtagggcgtctggctggagagctcggtgtgaggcagctcgttgtgggaagcgcggcgagcaggctcaccgtgcggggctgggccactgctgctctcactgaggaaacgtgggtcttcagggaccacgtggctttctgcgtttctcatttctagtactgtgcttctgaaaaggtgccagtctccaaaattcatattcatctctttcttcagctcatcaatgttacactgagctaacacacggccatttatgtttgcctttttgatcgtggtacaatactgaggcagcatactctggtccagcccttctatttgtttcagcttctcacatactgcatccacattcagtgaattcagtaataccactgggcctggggctgggcctgaccctaggccattgttctgatctctgggcaaactcgtttttactgatggacgtgagatgagatgttgggagccgccagggtaataccttggcgtgtaaaggtatggggcaaagaatggcctgttgtagaagggatgctgagggcccgtcatgccgctgtaatagctgctgtgaggctgtggtgacaccactccacctgcgaagggcccattgaaggacgtggaagagcacacggatgggggctggctgtaccctgatggcgccctaggaggaccctcatgtagagggagcggggggtacgccagtcctccaatactgatctgctctctggcagcacgaacatctgcaataatttcccgtagtttgggatctaggtttacagtgcatggcaaaaagacttttacatctcgagccacaagaactggggtccttgaagacaaaaacacttcaaaatttcttatatctccatcaatttcaagaagtggctcaacatccttagttgttggaatattctttgatattctttcgtagatggtttttaatgtcatttgatctggaataccttcagtctcttccaaatataatatgagccatgaagtccggtatggccactgctcagtaaggttgatccagctagcaagcctgtcccagttgaaactaatctgattggctctcagtaatcgtcctgtcacagaaacaatattaagtaatcttctcatggtctggggactgatgtcactgaaccagtcctcggtaaccagcagttttgtaagatcaaaggacatctggcgagtgatggtcctctgcatctgccttcttcggtaagtgtcccgtctattgagggctgtcttgctaccaagttttgtcatctccccaaggctgttctgtgaaactcttctgtcagcatcttcctgtatccctgtagtatctgagcatggaacgtctccatttgttgctgaagttacgagaaattttcttgcattgcttagtccacgactattaaggaacacaggcaagtggactatgttgcgcatgtagtcatggccatttatatttgaatcccgaagcacactattgaggttctggttaattgcctttatgataatatgtggatcacttgcaaaaatggcaatgaacgggccttttgaaaacagaactcggacagtgtccagcatctgaaggactttgtcctgctcacaggcatctaatccatcgatgatgaccaccagccttgtctgattctgagtgaagctgtcaatggtttttgccatcctggccatcaattccacttcacatttaagaactttcatgaatccttcacttttcaatttgtgcagtttggaggctgcattatggaggcgttttctttgggaattcaggagcgagtccagcacttgccaccatgtacgacagttcaacacaaaggccaatcccactacagatgcgattgatatgaggacagcatttacagtcagatgctttgggtcaactctaaatatagccagaagagtaattccagatataatgcagccaatgataaaaaggaagatgacaaaagatgggagacaacatgtttttttccatttctttttaccctgagtatcttcagtcttgaatactcgaaaaagcctggttgccaaaaagccaaactctctttcacaagcatccgagagggttgcaatcatttcagccagagaagtttctccacctacactggacagtctattgtaatctgtaaacaaaaacctcacaggtaaagctttagtagtctgctctggcaactcaggtggattcacaaacatcaatttaaggaggagttccaaatatccaatatgtcttgccaatctagtgctgaggacccaggcccaattccaactctctccttctcttcgtccaccaaagtaaatgacaataaagaatatatataagagagccaagaagctcagtgacactgctattccaagatttgggtggaccgtgaaggcaaacaataaaccaagccctccacaaagtagcagggtaagaaacactatgagccatgagaactgaaagagaggctcaatctgttgtccggcgaaggttttcatttcgtcttctagtttcttgagtaagaaagatttcccacttccccactgtgcatataaccccacacaaatgggtggctgcatggtaggctcactgagaatatctgccagggcactgctatataaatcatatccaagcatgtcaccgtctgtttcagtaggagacaagtgtctggctccaaatatttgagttaaaatactcttctgatggctacagtcaatattataaggagtctcgcctgctttgttgggcctataaagtaatcgcccatctttgggatttcttaaaagcagttctgccagtttccggctccttccacgaatagcaatatgcaagggagtatctcctttcttatctacagcagacactttagcacctttatctagcagcagctccaccacttcaatgtttctcatcttggtagcctttataagtggcgtttcaccatcctttgtgcatatttcagtgtcaggattgcactgtaagatatctctcaccattgttgcatttcctttctcaacagcccaatacaaagcagttttattatcctgtcctctaatgtctatatcagcatatttttggagaagcgctcgaacaatttcaacatgaccacctctgacagcgccaatcaacacagtatccccactcctgtcaggtatgttcacatatgttccagcgtcgagcagatcctgcacaatctccgtatgtccctcctttgatgcaatcatcaaagctgtatttccatctttatctgttaagtttacatttggattcctcttcaaaatttcttttactgactgtgtgtaacctcctttcactgccacaataagtgcagtcattgaattagctccttcttgatccacatcagctcccatggccaataaatgtttcacacattccaaatgaccctttcgtgcagcccaaactaaaggggtggttccatacttatcagagcagttgactttagcaccattttgcagtaaaagatgaactatatctgcatggcctctccctgctgcccaaatgattgggtaaacactgtacagaccagtgacacttggattggcaccatgagaaagaagcaactctactacgtcagtacggcctttgtaacatgcccacataagagctgtccatcctcccatatcacggtgctccaagttaaccccacatttcagtagttcctctacgatgtgcacatgcccttctttcgatgcagatataagtgctgtccaattatccaaatcttccagattgcagttagctccattcttaattaattccttcactatttccagattgccttgttcggcagctatcatcagtggagtctggccacactcatttctctcatctacatctttgcatttttcaagaagagctttcagagcaggaatgttttcttcctctacataatttatgacgctctgtgatatcaaaactgacattttcacagaaagctgcaattaactttatttgaatacctggtcctcagctccggcggaacgggcccgctcggctgcaggcgatgtcagaggacggggaagcaagagacggcgactgcaagcgcgtcgccctcaccacacccggcggccatattcttccctctccgcgaact

SEQ ID NO: 11019 - RNA, 552 nt, Homo sapiens
  source 1..552: mol_type = other RNA
ctgaatagctgggactacaggtgcacaccactaagctcaactaattttttcatttctttgtagagaaggggtctcgttatgttgcccaggctggtttcaatctcctggcctcaagtgatcctcctgccttggcttcccaaagtgctgagattatgggtgtgagccacatgcctgaccaggaatacactttaaaataataaagtatggtagcaacaggaaatggcaaggagtgcccctaatgttagctgactgcatgggttataattgtaatcattcatcgcatttttcgtctattagcaaatatacatgctctccatagatgatcacgtctgctcctcacaacagctttataaggtggattttaaagctcccattttatggaggaggaagctaaggctcagacggttttgattcatccaaggtcaaataggttgggtggcagaaccagaattccagccccgtgtgtcccttggctttgtgcctctgcggcgccccggagatctccttccccgtccctcttcctttccgagaagccgcgttccgttgttgaac

SEQ ID NO: 11020 - RNA, 3258 nt, Homo sapiens
  source 1..3258: mol_type = other RNA
ctgaatagctgggactacaggtgcacaccactacacctggctaatttttctatttttagtagagatggggtttcaccatattggtcaggctggtctcgaactcctgaccccaggtgacccacctgccttggcctcccaaagtgctgagattacaggcgtgagccaccatgcccggccctcaagatttttatgaggaccacatgaaatgctgaaagcacttagtagtatgtccaggagcagggtcttgctctgtcatctagacttgaatgcagcgagtggcatcgtcatagctcactgcaggctcaatctctcagcctcaagcaatccttgcccctcagcctcctaagtagctgggactacacgtccagctaatttttgtatttttgtaaagatggggcctcactatgttgccttggctggtcttgaactcctagtttcaagttatcctctcaccttggcctcccgaagtgttgggattataggcgtgagccactgcaactggccaggacagtgattgattgattgattgattggtttgagacagagtctcactctgtcgtccaggatggagtgcagtggcacgatctcagctcactgtaacctccacctcccgggttcaagcaattctgctgcctcagcctctcgagtaggtgggattacaggcacattccaccatgcccggctaatttttgtatttttaggagagacagggtttcaccatactggccattgctggtctcgaactcttgacttcatgatccgcccgcctaggcctcccaaagtgctgggattgacagtggcatttaaatagagaccttttagaaaagtgggaaagtagaaaaataaataataaatacataaatagagacctgtaaatgatgaacagtgaacttggtggagaagtgagatgggcatggggaggatagccctcaagcagagggaacagggtagaaatcaatcatgcaacaccaaattcaagcagtgaggatagaggggacagccaatcctctagggagggctaaggatttcctgactgataaagcctgagcggcaaagaagcctcctatccagccttgggcaagtctctgccaagctgggacttcacactacactggccagccattgacttccctgatagaaaaaccacaaccaacaagtcctcgctggggctggtctgccaaacacagaagacagagggaaggggagggggctgtcttggggtcagaagtgagcaggttttccaggggagaaggaagattgagaagaggggtatggctgctggctcacacctataatcccaacacttagggaggccaaggcgggaggcacacttgtggccaggagttcgagaccagcctgggcaacatagcgagacttcgtctgaacaaaaaaaaattatagtttaaaaattagctgggtgtagtggcgcgtgcctgaagtcccaggtattcacaaggctgagggaggaggatcgcttaagcccaggaggtcgaggctgcagcaaactatgatcctgcaactgcactccaacccaagtgacagagcaagaccttaaaacacacacaaaaaaaaccaaaaaacggcagaaagatgagaagccgttccatttgcataggcagttgaagtgtctaggcagaggcctccaaggctgactggatatcaggcaggggatgaggctggacagcctgcaatgcctccaactccaggttgcggaaatcgtgtttgtagtacctcagtcgaatggagattgagcgccccctgggagcagtgctcggtaacagacgctggaggaccccgatgaggaggggcgggggtcggttcaatctgggaggagcctgcgggtcagttttcttctcacaggagcgaactctgtccggcatcatggattcctgggctcccagaacggctgggctggaagggaccttagaaagggatctaccaccgcgtgccccgtgccagagttgggcactttggtgacaagaacattggcttgtttaacactcacaactgtgcttcgaggtggggatcattatccccattgtccccattttgcagatgagaaaaagcaaggtttggtggcttcccggggcggggcggggattcgctgtgactccaggtccttttccccggagcccgcacgtcttgtaagacactgattcccggaggtctgaggagcaggaatcgagtgggaggtgcccaggctttctagggaacaagagtgtgaatgcactctcgacgagaaccacgcccccctgttcgacaagactgattcctgctgccttcctttaagggccctcccctgaaacgcgaagtcctcgccccatggagaggcggacattctttattcccggatcgcccgacgtttttctcccccacccgcactgatccccactggtgacataaatccttcccctccactcgcgagtgaaagcttgggactacatttcccgccaggctgttcagaagccggtggcggagagaggagaaaagagtctttccgtttccgtcgcctcgcaatttggcgtgtccgccgggattcacatttcaacagcgacgtcctttctctgttggactcggcaaggaactacatttcccagcaggcaccggcgcagaggtcgaggggcgaggtcgccatctttttcgtagtcctctccctcatttccgcagggaagaggccagacgcctggactacacatcccatgtcgcagtcgccccggccctgcagccgccatctttgccggtggccccgccccatccccttccattgtctcgacttgagatgatagacgggagccgggagactgcaactcccgtcaggccgtgcgccactggtgggggggatttcgagaccacaggcgggcgaggtgcccaaggtggtggaaagcggagaccgggagaggctaggtagcctgccatctttacggtagtctcctcgtcctcctggttccgccattcttaaggaacactggaaggctataaaactactaatcccatcgcacctcgtaagatcgactactagtcaggtgtatgtccctcttccgccatcttgcttgtagtcctctttccttttcacctttccattgttcctgacgagtagaaatggcagcgggaaggcagcagatggactgcgactcccgtcaggtaccacacacgcggagggttgtggacaggagggcgtgtgagtgcctgggaaggaggtcgggtcgggggagaaggccatcttgtttgtagtcatcgttccctctccttctcgatgtt

SEQ ID NO: 11021 - RNA, 7341 nt, Homo sapiens
  source 1..7341: mol_type = other RNA
ctgaatagctgggactacaggtgcacaccactatgtgccccagctagtatatatatatatatatatattttgtatttttagtagagacgaggtttcgccatgttgcccaggctggtcttgaactcctgggctcaaagtgatccgtccgcctcgaccccccaatgtgttgggattgcaggcgtgagccaccgcgcccggccaaaatcttaatcctagtggaaaactgacagccccaaaaggttaataaatgtactcgaggctgacactgtataagacgacgacagattccatgatctgtatgactttggtcattaaatctgaactccttaaacctgcaattgaaaaagtagtataatcacgtctcatttctcttcagccaagactaatcttagatgtaaaaactgagaaaactcaggaagtccccacagcaagaattcagagtcatgacaattttggcaaaatcatcttctaatgccctgttaattaaaaaaaaaaaaaaaattcgcgcatcccgagacagtggtgctccccacatagcccaggtgggcaccgcatccaccccatgcctacacaggaggggactctctccatcctgaacttcttgctttggaaagttattgcttagtataaaaaatgagaggagtagggtggaactggcaatgaaggtcatttgctgcgcactctctggcaacgtccgcctgcattttgcactaggactcaacttccttccgtgtaccccaggcggcccctgcacgggtctggagagcaccccaggttgcgctggagtctggaaacatatcagcaccggaaaatatgttgggtgaagggtgagtatgaggggactgcaggcccaaggacccccgaaggaacggctgcctccccagcacagcacagccgcgctgcaccagccaccgaggacttccttatgtcagagcagaactcagggagggaggtgtgaggtcgcccatgaccacaggggctcgtgacgatgtgacgaagctacactgggagcactcgggccctttcaaagccagaagagaacctggggcttaatgcagaacggagggtccgtgagatgagtcccgggccatgcaggaccacccaaggccccgacccgaactatgtgtcggctgctgatgctctgccgtcggccgtcgtcccttgtccatcccccttcacagctgcaggatgtggtgttatctcatcccacatggataaccacagactggccaggcccagctggacgtgacgtggagtggctcggaggagaagattcggctgtggaggtttttttaaagctcaagtccccaccacctgaagtgtgcacacatcatcaagtcgaacggtcccccacggctggtatgctctgcggagatgagtctgcctgagttccccggcttcttgaaggaaggactgacaggaacacggaagcttcccagcagcctggcctccgaaaaccaggcagaagagctgcgcggagggaagcggtgcggtgccccgtgcagggtgcagctctctggacctgccacgccagcacgtccccagggatgggccgggtccatctgaggtctgcggccacaacctgttggtttttaccaaaagggctttaaaaaatgggatgtggggtgggagaatgacaaggagaggctgcaagacctctcagctcctcagagagaagcctcatttgctgcggcaaagccgcttcatcaagaagagacaaaaatgcattcaagtccatcaacaaaacagtggtattttggactcaatgaaaatatttcctatatgaacataaaacactaacattcagaatcatttatcatttatgaaagagtaccatatgtacaatcccaacaatcctagacacagtagaacactcaaaatatttaagcttcacaagtaccatgcagcgcaaactataaaacagaaaaaaaatcaaactagtggctagcatcggcttgacctgcctcattcccctcgaataactgaagatcctgtacaacaatggagactctcggaacatttatccacagtgcaattacagaaagcagttcgtgatttctctagaaataataaatatggctcactggtgaccattcccctcacgtgtcctctgtggtgcccacacgtgcgccgggatgtgcaggcgtggacgcagagacgcccctgtggaaagcacacatgcggtgcacacagctccacacgcgcgcgcacatggaggctgtgcccctgcctcccccgacggccagcgcatgagcactgcctgggaggccgcggccgcgggtgcacggggcactgagggacgccggctcctggacacggcctcgctctgcacctgggctcccgagggccccgccttgaacgcagctaagagccgtctccctcttcacctctggattcttcctcccaatctcatgtcagcaaatggcgagtggatgtcgctgctcgggctgagggcgcaggggcgccgctccaggggagcagcctcggacccgagcgtgcgcgttggcagccacctagtccttttctccgtcttcgctgcttccgccctgctcgatgtccgagtcggtcaggtgtgtgagggaaaagctggcaatgttggcgggagagatggagaaccgggagtaaggcgccgagtgcggccagctctgctccgtgctccgggccggtggcggcggagaaaagtacttggatgtttggagagaaggcttggagctgagcaggttacttgttgtctttgacataaaaggatctggggagaagtcatcatcccactcaaagccaccaccttcttcgtcggtggagctttcggagttgatgcacctgctcaggtagggagagcctgaggctggggctgggccgctcaggtccgggccgcacgcctctcctccacagggccccagctctttggttggggtctcctggtcaaacaggtagactgtgacatcatcgaaaaacgtgactgccttcttttccttcttccagtcctcgggcagtgggtcgggggcattggccgctgtgggcttcaacagactccgcaggtgccttccgtcctcgttgctgaggatgatgggcacggggtgctcggtctcgtcctccgactcggagctgaggctatgcaggttgaaggcccgcaggtcctcgtccgagtcgtcgctgttttcgtcctcctcgtctgcatccatcccgtcctctgagaggtcgagcatccctgacaccccgagtttccccaggtacttcccttcgatgtccggctccttcaacttcgggccctcggagtggctggacagggacttgtccagcgcagaattggtgtaggcaaggagttcgttcgtgttggtccccgtggaagcgagggtgcaggggcgatcgtcctgtgtctcgaagtcatcgccgctgctaagttctgcattcagcacactccagggactgctggcctcgtcttccgtgggatgcacctgctggggaacaccagtctgtgctggctccggcgtggctcttaattccaggtcactggagttgtgcaaagcagacagacaactttcatctggctggctctttctggcttccaggcagctatcctgggcagcaggactttgctcggggaggactggctcgggtaggggctgctcctgtaccaacaccaaggcggatggggaggttcccgggacctcctcagaccttttctcgggctcagagtcattgtctgagaagtacgcagagtctcggtatgaaccctgggagccagctgtgaacgtctcaggggtcacttctgtgcctctgtgaccatcgccggcatctgagatgacaatgaccgggttgggaggcagaccgctgtggccgccatcgcccgtggtggctggttctgagtctgcggtgccctcgggagcgggatgcaaggtccactcgggagactccaagttctctgtttcgtagccactgtctgccggcttatcggggggcactagtttctggggagtgtgagatcctaaagagtccagtagcgcttcgtggacatccactgactccagagagtccggggtttccagggacggctcagaggctgggaagggtgctgacaagctgtcctccaggaggctgtcctgactggttgagtccgaggagagggcagacaccaagcctgcttcttttgctgcgtctttagaattgagctgatttaaagtctccacagcctctaagtttttctctagccggcgatgactgtgatggtcttccgaaaatggtttattgtgcaattcctgtcccagttccgggagactactccctacactcaccctgctggcaaggatgtcatcagcaagaacagagtcactttcggtgagtcgcagggtctcctcactctcgccaggagagtcctgggacctgttatccaggctgtgggttctggcatcagttgagagaatttcaaccgggacagtcacagcgtctggactgatgtcctggtggagacagtcctccgggacaataacatctaaacacgtgggctgggtttctccctgtgttgggagtgagtctgggggtacccgacggggcgtttcttctgtttcgaaggaggtaggaggtacctgcacttccggggaagactgcaatgaggtgctcaaagtgtcacctgtgagcatgacatctgtatcgtcaccctttgtgcttacgttttcctgcaacaaagacaagcctggcttattttcagcaaactgaagctcagtatctaaagagtttctacatgacgtttctaacatagcttcagtaaaaccagcattcttaagttctgtctgaagatcatttatgtgttctttgctggacaatgagccttttagtaagtttttctcttgaagaaataaaaagttttctgacaattcttgaacattcaatggatcaaaattatcttggtgcataagattatctgataggcagagaggctcactgtcaaaaatcttacggggcttttctttctcaaagtggcctgttatgactgactctttggggttatccaaactggaacttaaagtggcaggtttaaagtcggcttgaactccgtttaattccattaagtcgaatattttttggtgactgggcaaatcttccgatttgtccacatcattaaatatattgttgaaagggctctcggggccactggtcacgtgtaagtcccctggtaagctagagtctttggggtctgtactgctttggaagaagtcctcatctgtactggactcctcaagttcaacgctcctgagcgccgtgagctgggacagttcagggccagtcctttctggattatccatgtcggttgtgagcagcgctggtgggtaatcaagctccaagttactaccacttttttcttctaactggatataatagtcgcttccaacagaaaggttgtgggcatcaaaaacaggaaccactccagggaccctcagggggacatcctggccgctgtcatcttgctttccgggcccaggatctgaaagcgaactctcaaaaacttcaaccggatagaagatgctcgtgtaggacaagccttcgtccaggtggccccggctgcgctcgtcaaagtggtcgtgcttagcggcctcccagacatactcgaagctcaggccctggctggtttcggtcacggtgaggacttcctccatttcacgacccagccggtccctggcaaagtggtcgagaattgggaatgcagcattgttggaggagtctctgctgtttgtgttcggcttcagagcgttccactgctgttcaaagtcgacctctgagtcccgctggctctgcagccgcaggtaagtcagcagcctgtgcacatcttcagccgcgggtctcttttctggtgacagccaacagaactgtaagacttcataccatctatcagagtagggctgctccagctggggcttcgggagttttgtgtctctctctctaatgacttggttgaggacatctaagttggaaaggtttgaatacggctgtgcggcattgtcaaaaagctcccaaagtgtcacacccagagaccagatattactatacttagtctgatctgcagttagcagtctgtcttgaaagctggttactaattctggagcagtccatcgcagagggaaaacttttttatcatctgtttcaatataatcctccttgtacctgctgaatcctattccgtaatctcccactttcacatttaagtcggaggtgagaaaacaattccgcagggctaaatcactgtgcaggaagtgcagcttgtgcatggcggccagccccgcggcgacctcgcacgccatcctctgcagcagcatggtctgtgagtccccccgcatgtgctcctgctcgctgcgcagatacgccttcaggtcacccaagtcacagaactcaaacaccaggaggtagggaatcgcttctacgcactgtccaacacactgaagaatatttggatgctgaagaatgtagtaaggttctccatttttcaaaaaagtatcttgttcctttgggttggcacttgcttttaactccttcacgatgactcttgctacgctagtgcccgtgtaaatctctcccaagagaacctttccaaaccagccatttccaatttcctgtatgtagtttagactgtggcgggcaacttgagacttcaatccctctacagaaggctggaattgcgagggagctgggagtgaaatatttggtactgaaagtgtgaagacctctgctggggactgaacagagggagtgtcttctgctggtggtgtgaaatctatctcatcatcaaaattatcttcaaattccttaaagtctatttctgggtccttacagcaggatacacagtttgcaattaacactattaatattattaaactgcacacacacaggatcacaaaagatgaggaaacttctgcagcaggtggcgcctcccctgcacctgtttgcggaagtggcgcggccccagcactgccggcgatcaggaggaccagcagcagcagcagcagcctccgccgcaacgccggcggccccggcatctcgcccacggcgcggctccggggccggccctcgagtcgccttccgtccgtccgtccgttcgcccgtcagtcgatcctgcctccctccgctgcctcagtggcacccgcgccggttgctcccgagcacacgttgcttctgccaaacctcggtccggctcccggtccgcacctgccgctccagtcgcagaaacaccatccttcccgcccgcctgcgccgccgccgccgcctctcaacagcagcaacgccagcagccctgcggagcggcgggcctgggaagccgcgctcccgccgccatgatgggctgcgtcatgtgac

SEQ ID NO: 11022 - RNA, 7329 nt, Homo sapiens
  source 1..7329: mol_type = other RNA
ctgaatagctgggactacaggtgcacaccactatgtgccccagctagtatatatatatatatatatattttgtatttttagtagagacgaggtttcgccatgttgcccaggctggtcttgaactcctgggctcaaagtgatccgtccgcctcgaccccccaatgtgttgggattgcaggcgtgagccaccgcgcccggccaaaatcttaatcctagtggaaaactgacagccccaaaaggttaataaatgtactcgaggctgacactgtataagacgacgacagattccatgatctgtatgactttggtcattaaatctgaactccttaaacctgcaattgaaaaagtagtataatcacgtctcatttctcttcagccaagactaatcttagatgtaaaaactgagaaaactcaggaagtccccacagcaagaattcagagtcatgacaattttggcaaaatcatcttctaatgccctgttaattaaaaaaaaaaaaaaaattcgcgcatcccgagacagtggtgctccccacatagcccaggtgggcaccgcatccaccccatgcctacacaggaggggactctctccatcctgaacttcttgctttggaaagttattgcttagtataaaaaatgagaggagtagggtggaactggcaatgaaggtcatttgctgcgcactctctggcaacgtccgcctgcattttgcactaggactcaacttccttccgtgtaccccaggcggcccctgcacgggtctggagagcaccccaggttgcgctggagtctggaaacatatcagcaccggaaaatatgttgggtgaagggtgagtatgaggggactgcaggcccaaggacccccgaaggaacggctgcctccccagcacagcacagccgcgctgcaccagccaccgaggacttccttatgtcagagcagaactcagggagggaggtgtgaggtcgcccatgaccacaggggctcgtgacgatgtgacgaagctacactgggagcactcgggccctttcaaagccagaagagaacctggggcttaatgcagaacggagggtccgtgagatgagtcccgggccatgcaggaccacccaaggccccgacccgaactatgtgtcggctgctgatgctctgccgtcggccgtcgtcccttgtccatcccccttcacagctgcaggatgtggtgttatctcatcccacatggataaccacagactggccaggcccagctggacgtgacgtggagtggctcggaggagaagattcggctgtggaggtttttttaaagctcaagtccccaccacctgaagtgtgcacacatcatcaagtcgaacggtcccccacggctggtatgctctgcggagatgagtctgcctgagttccccggcttcttgaaggaaggactgacaggaacacggaagcttcccagcagcctggcctccgaaaaccaggcagaagagctgcgcggagggaagcggtgcggtgccccgtgcagggtgcagctctctggacctgccacgccagcacgtccccagggatgggccgggtccatctgaggtctgcggccacaacctgttggtttttaccaaaagggctttaaaaaatgggatgtggggtgggagaatgacaaggagaggctgcaagacctctcagctcctcagagagaagcctcatttgctgcggcaaagccgcttcatcaagaagagacaaaaatgcattcaagtccatcaacaaaacagtggtattttggactcaatgaaaatatttcctatatgaacataaaacactaacattcagaatcatttatcatttatgaaagagtaccatatgtacaatcccaacaatcctagacacagtagaacactcaaaatatttaagcttcacaagtaccatgcagcgcaaactataaaacagaaaaaaaatcaaactagtggctagcatcggcttgacctgcctcattcccctcgaataactgaagatcctgtacaacaatggagactctcggaacatttatccacagtgcaattacagaaagcagttcgtgatttctctagaaataataaatatggctcactggtgaccattcccctcacgtgtcctctgtggtgcccacacgtgcgccgggatgtgcaggcgtggacgcagagacgcccctgtggaaagcacacatgcggtgcacacagctccacacgcgcgcgcacatggaggctgtgcccctgcctcccccgacggccagcgcatgagcactgcctgggaggccgcggccgcgggtgcacggggcactgagggacgccggctcctggacacggcctcgctctgcacctgggctcccgagggccccgccttgaacgcagctaagagccgtctccctcttcacctctggattcttcctcccaatctcatgtcagcaaatggcgagtggatgtcgctgctcgggctgagggcgcaggggcgccgctccaggggagcagcctcggacccgagcgtgcgcgttggcagccacctagtccttttctccgtcttcgctgcttccgccctgctcgatgtccgagtcggtcaggtgtgtgagggaaaagctggcaatgttggcgggagagatggagaaccgggagtaaggcgccgagtgcggccagctctgctccgtgctccgggccggtggcggcggagaaaagtacttggatgtttggagagaaggcttggagctgagcaggttacttgttgtctttgacataaaaggatctggggagaagtcatcatcccactcaaagccaccaccttcttcgtcggtggagctttcggagttgatgcacctgctcaggtagggagagcctgaggctggggctgggccgctcaggtccgggccgcacgcctctcctccacagggccccagctctttggttggggtctcctggtcaaacaggtagactgtgacatcatcgaaaaacgtgactgccttcttttccttcttccagtcctcgggcagtgggtcgggggcattggccgctgtgggcttcaacagactccgcaggtgccttccgtcctcgttgctgaggatgatgggcacggggtgctcggtctcgtcctccgactcggagctgaggctatgcaggttgaaggcccgcaggtcctcgtccgagtcgtcgctgttttcgtcctcctcgtctgcatccatcccgtcctctgagaggtcgagcatccctgacaccccgagtttccccaggtacttcccttcgatgtccggctccttcaacttcgggccctcggagtggctggacagggacttgtccagcgcagaattggtgtaggcaaggagttcgttcgtgttggtccccgtggaagcgagggtgcaggggcgatcgtcctgtgtctcgaagtcatcgccgctgctaagttctgcattcagcacactccagggactgctggcctcgtcttccgtgggatgcacctgctggggaacaccagtctgtgctggctccggcgtggctcttaattccaggtcactggagttgtgcaaagcagacagacaactttcatctggctggctctttctggcttccaggcagctatcctgggcagcaggactttgctcggggaggactggctcgggtaggggctgctcctgtaccaacaccaaggcggatggggaggttcccgggacctcctcagaccttttctcgggctcagagtcattgtctgagaagtacgcagagtctcggtatgaaccctgggagccagctgtgaacgtctcaggggtcacttctgtgcctctgtgaccatcgccggcatctgagatgacaatgaccgggttgggaggcagaccgctgtggccgccatcgcccgtggtggctggttctgagtctgcggtgccctcgggagcgggatgcaaggtccactcgggagactccaagttctctgtttcgtagccactgtctgccggcttatcggggggcactagtttctggggagtgtgagatcctaaagagtccagtagcgcttcgtggacatccactgactccagagagtccggggtttccagggacggctcagaggctgggaagggtgctgacaagctgtcctccaggaggctgtcctgactggttgagtccgaggagagggcagacaccaagcctgcttcttttgctgcgtctttagaattgagctgatttaaagtctccacagcctctaagtttttctctagccggcgatgactgtgatggtcttccgaaaatggtttattgtgcaattcctgtcccagttccgggagactactccctacactcaccctgctggcaaggatgtcatcagcaagaacagagtcactttcggtgagtcgcagggtctcctcactctcgccaggagagtcctgggacctgttatccaggctgtgggttctggcatcagttgagagaatttcaaccgggacagtcacagcgtctggactgatgtcctggtggagacagtcctccgggacaataacatctaaacacgtgggctgggtttctccctgtgttgggagtgagtctgggggtacccgacggggcgtttcttctgtttcgaaggaggtaggaggtacctgcacttccggggaagactgcaatgaggtgctcaaagtgtcacctgtgagcatgacatctgtatcgtcaccctttgtgcttacgttttcctgcaacaaagacaagcctggcttattttcagcaaactgaagctcagtatctaaagagtttctacatgacgtttctaacatagcttcagtaaaaccagcattcttaagttctgtctgaagatcatttatgtgttctttgctggacaatgagccttttagtaagtttttctcttgaagaaataaaaagttttctgacaattcttgaacattcaatggatcaaaattatcttggtgcataagattatctgataggcagagaggctcactgtcaaaaatcttacggggcttttctttctcaaagtggcctgttatgactgactctttggggttatccaaactggaacttaaagtggcaggtttaaagtcggcttgaactccgtttaattccattaagtcgaatattttttggtgactgggcaaatcttccgatttgtccacatcattaaatatattgttgaaagggctctcggggccactggtcacgtgtaagtcccctggtaagctagagtctttggggtctgtactgctttggaagaagtcctcatctgtactggactcctcaagttcaacgctcctgagcgccgtgagctgggacagttcagggccagtcctttctggattatccatgtcggttgtgagcagcgctggtgggtaatcaagctccaagttactaccacttttttcttctaactggatataatagtcgcttccaacagaaaggttgtgggcatcaaaaacaggaaccactccagggaccctcagggggacatcctggccgctgtcatcttgctttccgggcccaggatctgaaagcgaactctcaaaaacttcaaccggatagaagatgctcgtgtaggacaagccttcgtccaggtggccccggctgcgctcgtcaaagtggtcgtgcttagcggcctcccagacatactcgaagctcaggccctggctggtttcggtcacggtgaggacttcctccatttcacgacccagccggtccctggcaaagtggtcgagaattgggaatgcagcattgttggaggagtctctgctgtttgtgttcggcttcagagcgttccactgctgttcaaagtcgacctctgagtcccgctggctctgcagccgcaggtaagtcagcagcctgtgcacatcttcagccgcgggtctcttttctggtgacagccaacagaactgtaagacttcataccatctatcagagtagggctgctccagctggggcttcgggagttttgtgtctctctctctaatgacttggttgaggacatctaagttggaaaggtttgaatacggctgtgcggcattgtcaaaaagctcccaaagtgtcacacccagagaccagatattactatacttagtctgatctgcagttagcagtctgtcttgaaagctggttactaattctggagcagtccatcgcagagggaaaacttttttatcatctgtttcaatataatcctccttgtacctgctgaatcctattccgtaatctcccactttcacatttaagtcggaggtgagaaaacaattccgcagggctaaatcactgtgcaggaagtgcagcttgtgcatggcggccagccccgcggcgacctcgcacgccatcctctgcagcagcatggtctgtgagtccccccgcatgtgctcctgctcgctgcgcagatacgccttcaggtcacccaagtcacagaactcaaacaccaggaggtagggaatcgcttctacgcactgtccaacacactgaagaatatttggatgctgaagaatgtagtaaggttctccatttttcaaaaaagtatcttgttcctttgggttggcacttgcttttaactccttcacgatgactcttgctacgctagtgcccgtgtaaatctctcccaagagaacctttccaaaccagccatttccaatttcctgtatgtagtttagactgtggcgggcaacttgagacttcaatccctctacagaaggctggaattgcgagggagctgggagtgaaatatttggtactgaaagtgtgaagacctctgctggggactgaacagagggagtgtcttctgctggtggtgtgaaatctatctcatcatcaaaattatcttcaaattccttaaagtctatttctgggtccttacagcaggatacacagtttgcaattaacactattaatattattaaactgcacacacacaggatcacaaaagatgaggaaacttctgcagcaggtggcgcctcccctgtttgcggaagtggcgcggccccagcactgccggcgatcaggaggaccagcagcagcagcagcagcctccgccgcaacgccggcggccccggcatctcgcccacggcgcggctccggggccggccctcgagtcgccttccgtccgtccgtccgttcgcccgtcagtcgatcctgcctccctccgctgcctcagtggcacccgcgccggttgctcccgagcacacgttgcttctgccaaacctcggtccggctcccggtccgcacctgccgctccagtcgcagaaacaccatccttcccgcccgcctgcgccgccgccgccgcctctcaacagcagcaacgccagcagccctgcggagcggcgggcctgggaagccgcgctcccgccgccatgatgggctgcgtca

SEQ ID NO: 11023 - RNA, 634 nt, Homo sapiens
  source 1..634: mol_type = other RNA
ctgaatagctgggactacaggtgcacaccactgtgcctggttagttttgtttattttttgtagagacaaggtctcgctctgttgcccagtaaaatcaggtctttaatacaaatgttctgactcccatgcagaattctttcctgttggcacgcaaactcaacactgcagtagaagcgtgggctttacggttatcacgacgtgccaataaatcctgcgttcttcatgttcaatgctggaaccttggacataattcctcaagtcttggtatgtttaactggacctcctggtgacaccaagaaggagtctaatttcaccaccaccaggttttttgttcacttgttcagcaaatatttagggagcatacaatgattaaagagtaaacatggttcctgctgtcttggagatgactttgctccagtttatgggtgaggaaactgaggcccagagaaggtcaatgacttggccttgttcatccagatggcgattgaaggggaaggaattgagactttgctgggcttggctccaaaacaaagactgcttccaggccattatgctgtagatctctggtacaggatgatctatagggcagacctttccttgtgggctgggatcttgctcatggcagcagttgctt

SEQ ID NO: 11024 - RNA, 12890 nt, Homo sapiens
  source 1..12890: mol_type = other RNA
ctgaatagctgggactacaggtgcacaccatcacagctgactaatttttcttttctttttttttttttgagacggagtctcactctgtctcccaggctggagtgcagtgatgtgatctcagctcactgcaacctacgtctccagggttcatgtgagtttcctgcctcagcctcctgagtgagtagctgggattacaggcgcctgccaccacgtccagctaatttttgtatttttagtagagattgggtttcaccatgttggccaggctggtctccaactcctgacctcaagtgatccacctgcctcggcctcccaaatcgctgggattacaggcgtgagtcatcatgcctggccttttttttttttttgtgagacagagttttgctcttgtcacccaggctggagtgtaatggcatgatctcggctcactgaaacctctgccaggcacacgtcaccatgcccggctaatttttgtatttttggtagaaacggggtttcaccatgttggccaggctggtctccaactcctgacctcaagtgatcctcctgccttggcctcccaaagtgctgggattacaggtgttagctaccaagtctggcctttttttttttttttttttttttttttttttgagacagagtttcgctcttgtcacccaggctggagtgtaatagtgtgattccagcttactgcaacctctgcctctcgggttcaagccattctcctgcctcagcctcctgagcagctgggattacaggcacacgccagcatgcctggctaatttttatatttttagtagagacggggtttcaccatgttggccaggctggtctcgaactcctgacctcaggtgatccatctgcctcagcctcccaaactgctgggatgacaggcgtgagccaccacgccaggccctatttttatttttaaccagtgctgtagtttgaatatttgtctcctccaaaactcatctggaaacatccccaatgtggcaatattgagagatggcgcctttaaaaggtgactgggtcatgaaggctctgcccagtgagactggtgcctttataagaagaggaagagagacctgagctaccatgctcaagtccctcaccacgtgaggccctctgccaccttgggtctctgcagagagttcccaggaacaagaagtctctcaccagatgtggaccctgtaccttggacttctcagtctccactattgtaagaaataaattccttttctttataaatgacccagtttcaggtattctgttctatgcaacacaaaatggactaagacaacgagtacgcttagttgttgcttcctgagttccaaagtccgacagacagagcaggtcctccattcttgcccctttttaccccaaatgctcattggcattcttgcagctacgagtaataattaaaagtggctaagccaggctggcatggttgctcacgcctgtaatatcagcactttgggaggctgaggcaggaggatcacttgaacccaggagtgagaccagccagggcaacatagcaacaccctgtctctaattattattatttttttaagtgagtaagccaaataggggtttacttttcatctagaacaagaagacgtgttggccaggctggtctcaaactactgggctcaagtgatccacccacctcagcctcccaaagtgttgggattatgcgtgagccaccgcacctggccacaagacccaatttcttttattttatctttttttttttttttttaagagatagggcatctaacggcattgttttagctgctcaacacttttttttttttgcttatttttgtttgttttgtttgtttttgagacagggtctccctctgttgcccagcatatagtgcagtggcatgatcatggctcactgcagcctcaacctcccaggatcaggcaatcctcctgcttcagcttcctgagtagctgagaccacaggtgcacaccaatatacctaatttttttttttttgagatggagtttcactcttgttgcccaggctggagtgcaatggcgtggtctcagctcactgcaacctctgcctccctggttcaagcgattctcctgtctcagcctgccgagtagctggggttacaggcataagccactacgcccagctaattttgtatttttagtagagacagggtttctccatgttggtcaggctggtctcgaactcctgacctcaggtgatccacccacctcagccttccaaagtgctgagattgcaggtgtgaaccactacgcctggccacctgactaatttttaagttattcacagagaacaggttttgcaatgttgcccaggctggtctcaaactcctgggctcaaatgatcctcctccctcggcctcccaaagtgctggggttacaggtgtgccactgtgcctggtcggctcaccactttcagatctggctctcttcacctctcttttatagtcataagctgattagcacaattctagacatccgcagctacatttaaggcaggaaggaggtggtaatagacactaccagccacatctgtcccttttaatcaggataccctagaaatcctcagcagactttgaattatgtgccattggtgaaatgtcatatgatcatccctctacaaggcaacgaggtaaaaagagaatttagtatttctagcctctagagtggagatgaacaaagaataggaatgggcatttgcttaggaaaccaactgtgccttacaacatttttgcacttttttctgtaacattttgtgttaaatcatataaaaatgctgatcctaacaaatatggtcaatgagtcacaccataattctctaagaactccagtccaaaaaggttaatcttgcttttaaactccaggcgcggtgtttcacagctgtaattttagcacttcgggaggcagagcaagaggatcacttgaggccaggagttggagaccagcctggcaacatagcaagaccccgtctctacaaaaaataaaattatctgggcctgttggtgcacacctgtagtcccagctactcaggaggctgaggtgggaggatcacttgagcctaggaattcgaggctgcagtgagctgtgattgcaccactgcactccagcctgggtgacagagggagaacctatctccaaaacaaaacaaaataaaaacaaaacaaaactccaagcagagaaagacttgacgagtcggatgagtctgatgattcctaaaggaaatcctttttgagattccaggagattccatctcctcaacagagtaattgattttgagcctcccacctcctgaattaaggcccacccatccctatcctgcactgaactgtagactcttttttacttccttacaaaagtttattcttaaatgtacaacagactccaagacgacactttattgtagctataggtggcaaaagatgttatggcagagaatccagatgtttaaataggaatggggtcaagggtcaccgccccaagcacggataacaaaatttattttttgccagatttctttaattccacctgtgactggtgagggctggtggcggggtggctttcacttttagctcctctttttgtttctgcttgaacgtcccatcttccttacccacccccttgacctgcttcttgagctttctcagggcttcttgccacctttgcagctgtacatggcacctgccatagggctctaattttaaactgagaaattgagaaaacaggaaactgactctttttggggggagagtaagacaaacaggaaaaggaaaatgaagacgtggttgatacagatcgttggatttcaaaaggaaaagtctacggataaccgaaaaaaataaatatttagaaatgcatagtcttggctggttaaataagtatccatgcttgttcttgtggcatagtagttacgagacatttttagttaaatggaaaaatgtgaattactatagtttgagtgatatgctgctttccaaattaaaagcagcataacaaaaacattcccctaatactcataaataattcattgaattggcaataattcacctcctaatgacttcatatgaagtataaagtaacttcgatacatcagaagaaatcctatcttctaatataagaaagtaatatgattacattaaatgcgtctcatataagttataaaaatggtatctatgagtaaagaaatgcttgtgaacaaaaaaattgatcttataaaggtcaaacaggccaggcgtggtggctcacacctgtaatcccagcactttgggaggctgaggtgggcggagtacctgaggtcaggagttcaagaccagcctggccaacatggtgataccctgtctctacaaaaatacaaaaaattagctgggcatgatggtgggtgcctgtaatctcagctactcgggaggcagaggcgggagaatcgcttgaacccgggaggcggaggttgcagtgaactgagattgagccacaacaaccaagcctgggagacagaggaaactctgtctcaaaaaataaaaaataaaaattaaaattaaaaaaaaggtcaaacaaaccaaacccttctgattaatttattcaatctacttttattataagcaaatgagaaattataattttaatctgaaaaagcagaatcaggggattttggagctggacagtcccctggaaattatttggatcaaagccctcattttataggtgaagaaactgagaagtaagatttgagcaagctgcccaaaggctttgccaaaggctataccagtgaatggcagagtctggactggaagtcccagtgctgccgtccaggtgagacctgttccactgcatgctactagctcccgggctgagaccggacttttgcttggcaggtttctttctttcgaaactattaattattgtattttttgtagagacagggttttgccatgatgcccaggctggtcttgaactcctgagctcaagagatccacccagcttggcctctcaaaaatgttgggattacaggcataagccacagtgcccggcccattttcctcccacctctttgttccttctctgtttcttttgcagcattatgttctatcattgtataccagagttcctcaacttcagttatagtctgttcttgctttatgctatcttcttcagcaagctcatcttggtctgttttcctccttatcaggcataccccagaaactcctgttttatctccacctcaactaaacattttcctgagttctgggcctctataaactaattatttgattaacatcttttttttttttttctgagatagagtctctctctgtcacccaggctggagtgcagtggtgcaatctcagatcactgcagcttctgcctcccagattcaagcgattctcctgcctcagcctcctaagtagctgggattataggcatgcaccaccgcacacagctaatttttgtacttttagtagagacggggtttcaccatgttggtcaggctggtctcaaactcctgatctgaagtgatctgactgcctcagcttcccaaagtgctgggattacaagcctgagccaccatgcctggccaacatctttaattggatatctcagtatcaagaaggcccataatattcctctgcctcatccctctcctcagtcctcttcttgtgtttcctagttcagagaatggcaccattctctatcaagctgcgcaaatcagacatgtgtgattttttgttgttgttgagacagggactcactctgtcacccaggctagagtgcagtggcgtgatcatggcgcactgaagcctcaaactcctgggctcaggagatcctcccgcctcagcctcctgagtagctgggaccacaggcccacaccaccatgcccagctaattttgtattctttgtagagatggggtttcatcatgtttgcccaggctggtctcgaactcctggactcaagcaatccacccacctcagcctcccaaagtgctgggattacaggcatgagccactgtgcccagctgaagtgtgatccttaacttcaccccttctcatgccctccatttccaatccatctccagtccagttgactccagctactcaattatttccacttatctcattccactacctttgaagctaccaccatctctaactacagtcatctcccaactaactggtctcctggcatctctctggttctcctccactaatttcaaaaaaagaaatttactgtgacagtgctcacaacactcccccttgctcttactaaagatgcttaccatagcctccaggtattgtatggcctgaggtctatctacatttccaggtgcaggacacaccatgtctccccactcccaaatttagtctccagactccatcctttttacagttctttaaaagcatcacaattcctccaaccactaggcatttgtatgtgctattccctctttccagaatgcaataccctccctctgcctagctagctaacttctatgtatctatgactgcagctcaaactttcctcatggactccctccacaagtgccaagcctgggccagattcttttgttatgtgctcacagaacgatgttccctttagcattcattgagtttgctgtttaattattcttgtcttgtttttgtttaattagtcctatctctaatactagacaaatgttccttaagatcacaggaaatataggactgtctctacataaaaactgttttatatccataatgcctaggacagtacctggcacacagtatatgctcaataaatttttgttgaatgaatgcaattatcattatattcctgatattagcaggtataatccagtttaagtttgggaacagaaagacaaaacggaccacatctaataaatccggtctcctttcttttattatttatttatttgagacagttttgctcttgttgcccaggctgcagtgcaatggcatgatcttggctcactgaaacctccgcctcccaagttcaagggattctccagcctcagcctcccaagtagctgggattacaggcatccaccaccacgcccagctaatttttttgtatttttagtagagatggggtttcaccatgttggccaggctggtctcgaactcctgacctcaggtgatccacccacctcagcctcccaaagtgttgggattacaggcgtgagccaccgtgcccggccaaggtctcctttcttttaatcaaactctcacctttggccattctgcagtcattcacccgacagtatttactgacggagtgaatacagagtgcttgattaatgttgctgctttgttattattattattattattgagatggagtcttgctctgttgcccaggctggagtgcagtggcgtgatctcggctcactgcaacctccgcctcccgggttcaagccattctcctgcctcagcctcccaagtagctgggactacaggcatgcaacaccacacctggctaatttttgtatttttagtagagacaaggtttcaccatattggccaggctggtcttgaactcctgacctcaggtgatctgcccacctcagcttcccaaagtgctgggattacaggcgtgagccaccatacccaacctaatgtttctgctttgaaatacaatttcaaaaagtcattaataggttgaaaacagcaagattttaaaagtattttaaaaagtgaaacagaagaatgcttacttcatttcacagagatagatttctcctttatgttatttctaaaaggagatggaattttgtttcattcatttctgcttatttggacaggccaaatatgaacagctgaacacgtcagcgttaccatgcatatgttacacagatgccatccttcttccatcagctctcatatgcaatacagaagtaaaaagaggttctctttatttttaaaaggtaaaaattgaaattcagtcacttaacacagaataaacaataattacaattacactggtaacaaaggacagcaagcatgttttctttgaaagcactgtatctggtttgtctccgtgcttggtcctagtatctggcatattttccccagagttttcttttcagtgggatgattatcttcggggcaaaaaagtttatcagactcaagttttagcagtacttattttattcatttatatacatgtaaccccatcctgtcttactccaatcttcttactgccttcctactgacacatatattatataacaccctccccaagttctatttacggttaaaaatttctttttttttttctttttttgagacagagtttcactctcgtcacccaggctggtgtgcaatggcgcagtctcggctcactgcaacctccgactccctggttcaagtgattctcctgtctcagcctcccgagtagctggaattacaggcgcccgccaccatgcccagctaatttttgtatttttagtagagacagtgtttcgccatgttggccaggctggtctcaaactcctgacctcaggtgatccacccgccttggcctctcaaagtgctgggattataggcgtaagccactgcgcccagcctacagttacgaatttctaaatggcacaaataaactcagctgttctcagtgcagacgtcaaatcctcactgtgctgaaacattttcctcagcttttgggaaataattacaatttaaacatacacagagaatgtttcttagacaaacataatacccgaggcttatctggtaaaaactaattgctctgtccttagcacaaaaaatatatatctttgtaaaatgagaagaaccaaagaatatttaaaacaaagaaggaagccacacgtactaattacacaagagactgactgacaaactggaattctccaaaacagattttcagcgaggcttctcatttcagagtccaggaaaaaaaaatcctaaaaaccccaaaggtatattatatgtgtgtatatatatttttattgtgttaaaaaacacaaaacataaaatttactgtcttatcaaaaggtatattttgtcgctcttccctttttttttttttttttttcccgagacagagtccagtctgtcgcccaggctgaagtgcagtggcatgatctcggctcactgcaacctgcatcttctgggctcaagcaatcctcccacctcagcctcctgagtagatggagctacaggcacgtgccactaggcccggctaatttttgtattttttgcagacagggttttgccatgttgcccgggctggtctttgttctcctaagagttgttttctccatgaaagttgataaataacatttagaaaatgaattattacaagagtaatgatatgtctcaatttattatatgaaattatcaacaactgcttttaatattcagatgtcaagaagatgaaaagcagaaatacattttgcaaacatgtagcactccataaatggaaatcatgtatttcctctaatatcccaatttttctatattgggatcttatatggctgtttctatatggctattttgtcccaacttgctgtacaagaattttccccagccaccttagaaaggttggatgtagttcactccaagtttgcagttcactccaagtgtttcagtaccacagaaagctccatggaagcctcaaatgtacgggctaggcaatagaagcagggaggtaggattaagaaattactggccaggtgtggtggctcaggcctgtaatcccagcacttcgagaggctgaggcagacagatggcttgagctcaagagtttgagatcagcctgagcaacatggcaaaactctgtctctacaaaaaatataaaaatcagccaggtatgttggtgtgcacctgtagtcccagctactggggaggttgaggcaggaggattgcttgagcccaggaggctgaggctgcagtgagccatgattgtgccactgcattccagcctggtcgactgtaagacaaaaaataagaaaataaaaaatttaccaatataaaatgctcaaacagctaacaaacatgttcaattccatttatagtcttttctttgagccatttaaacatagggctattttttttttttttttttgagatggagtttcactcttgttgcccaggctggagagcaatggcatgatctcggctcaccacaacctctgcctcctgggttcaagcgattctcctgcctcagcctcccgagcagctgggattacaggcatgtgccaccatgcctggctaattttgtatttttagtagagacgggattcctccatgttggtcagactggtcttgaactcccaacctcaggtgatctgcctgcctcaaccttccaaagtgctgggattacaggtgtgagccactgagattggctgccgttttgttttttaactccatatagtttctatagttcactgaaaactcaaagagatgacctataaatgtatgaataatgtatgatttcttacatcaattttctactagaaaaaaatcatacttttagaattggattttgtcttacagtcatctttattatactttataaatgagatttcatttatataaatcaggaagctaaactaaaatagaaacactagatttaaattctgatttgaatactctgatcaaaataacaaatctcacactgggaaaccatctatcagcaagcagagagctactgtgtgtccttccttagaagagtttgaacaccgagaacccacagcatatttgcagtacagtaacagcaattcctttgtcattatcacagaactttaattttcatatactttgctgggaccaaccaaaccatcccatatatataaccatatccatatatatatatatatatatcccacatatatatgggatggtatatatatacacatgtatatgtatgtgtgtgtgtatatatgtgtatatatgtatacacacacacacacacacatatatatatatatacacacacacacatatatatatggagagagagagagagacagtgtcttgctctgtcgcccaggctggagtgcagtggtacgatcttggctcattgcaacctccgcctcccaggctcaagcgattctcatgtctcagtctcccaagtagctgggattacaggtgtgcaccaccacaccaggctaaccattccatacattttatacaatcatttttaaaaagaagcatgaaccatttcggttttagagaattaagtttttttaaaaaagagactcttaaaaaaaagtcattatatgaataaaatctgctttgtgttaattccgacaaatcattccatcattgagtctgtcaccaattttttttttttgaaatggagtttcgctcttgttgcccaggctggagtgcaatggtacgatctcggctcactgcaaccgccgcctcccgggttcaagtgattctcctgcctcagcctcccgagtagctgggattacaggcatgcgccaccacgcctggctaattttgtattattagttgagacagggtttctccatgttggtcaggctggtctcgaactcctgacctcaagtgatccgctggccttggcctcccaaagtgctgggattacaggcgtgagccaccgtgcctggcccaattttttttttttaataacttgcacacttaacaatattttttatcttcttgggacaacattcttttctccacaaaaacccaattaaggacgttgtgccagtttactcctacttccttcctgttcactgagcttaaagtgggtataggcgagaatgccaaataatgtacataaaatgccaagggcctgattaatggacagtggatccttaaataaaacatatcctccgaataaagtaatgcagaacttgaagtgtccgaacatgttataggtgacaggtgaagtgttcccaatgatccaataaattgataagttcaccatgaaagctattactccagatagcagcaccataagcaaagcagaaactgaccagggaccaaatattcctccttctccaaacactggctcaaagaagggcacagcaaccagcaacatggcagatgacatcggagcctggtagtacagcagctgcattgagttcacttgtaattcatgctgtttggctcctacccaaaacaggtaggtatttggtgagcatcacacacccaagtttctctgtctcctttcttctcttcaccttgagtcagacaacttatgcaattatgctttcttcccaacagtctattgtctctatactgtattttctaaaccttggaatacagcttcaaaatttatgaaatcagcgtgagctggattctggtggagaaggttttctggtagcagaaggtctggatggctatgatcaccggcgtggtcatggccttggccagctgataggtgcctatggtgttgttctgcagagaaaggttagtgaagaccacaaagccacagaagctgagggccaggaggaggagcctggagggcggcagacttttgggggcaaagatgtccagcttctggcagatatacaagcccagccaggtgaccacgaagtgcaccagggtcaggctcatgttggggaagccgtggtacacataaatccatttgttgaggaacacaatgcagatggacaccagcaggttgaacaggagcccggcggcgattcgccagtggccccgcactcggtccaccagcaatgccatgatccccgcgaagctggggccgtctagcctcggaaggggcgccgggcctgtctccggctgcccttctactccaccgccgcgtcctcgcagacgccgacctcaccgtctgacccaggagtggcatgcacagatcaaccccgggcgagtagcactcttaacagaggacacacaccccgccgccgccctgtaagccagctaggac

SEQ ID NO: 11025 - RNA, 12893 nt, Homo sapiens
  source 1..12893: mol_type = other RNA
ctgaatagctgggactacaggtgcacaccatcacagctgactaatttttcttttctttttttttttttgagacggagtctcactctgtctcccaggctggagtgcagtgatgtgatctcagctcactgcaacctacgtctccagggttcatgtgagtttcctgcctcagcctcctgagtgagtagctgggattacaggcgcctgccaccacgtccagctaatttttgtatttttagtagagattgggtttcaccatgttggccaggctggtctccaactcctgacctcaagtgatccacctgcctcggcctcccaaatcgctgggattacaggcgtgagtcatcatgcctggccttttttttttttttgtgagacagagttttgctcttgtcacccaggctggagtgtaatggcatgatctcggctcactgaaacctctgccaggcacacgtcaccatgcccggctaatttttgtatttttggtagaaacggggtttcaccatgttggccaggctggtctccaactcctgacctcaagtgatcctcctgccttggcctcccaaagtgctgggattacaggtgttagctaccaagtctggcctttttttttttttttttttttttttttttttgagacagagtttcgctcttgtcacccaggctggagtgtaatagtgtgattccagcttactgcaacctctgcctctcgggttcaagccattctcctgcctcagcctcctgagcagctgggattacaggcacacgccagcatgcctggctaatttttatatttttagtagagacggggtttcaccatgttggccaggctggtctcgaactcctgacctcaggtgatccatctgcctcagcctcccaaactgctgggatgacaggcgtgagccaccacgccaggccctatttttatttttaaccagtgctgtagtttgaatatttgtctcctccaaaactcatctggaaacatccccaatgtggcaatattgagagatggcgcctttaaaaggtgactgggtcatgaaggctctgcccagtgagactggtgcctttataagaagaggaagagagacctgagctaccatgctcaagtccctcaccacgtgaggccctctgccaccttgggtctctgcagagagttcccaggaacaagaagtctctcaccagatgtggaccctgtaccttggacttctcagtctccactattgtaagaaataaattccttttctttataaatgacccagtttcaggtattctgttctatgcaacacaaaatggactaagacaacgagtacgcttagttgttgcttcctgagttccaaagtccgacagacagagcaggtcctccattcttgcccctttttaccccaaatgctcattggcattcttgcagctacgagtaataattaaaagtggctaagccaggctggcatggttgctcacgcctgtaatatcagcactttgggaggctgaggcaggaggatcacttgaacccaggagtgagaccagccagggcaacatagcaacaccctgtctctaattattattatttttttaagtgagtaagccaaataggggtttacttttcatctagaacaagaagacgtgttggccaggctggtctcaaactactgggctcaagtgatccacccacctcagcctcccaaagtgttgggattatgcgtgagccaccgcacctggccacaagacccaatttcttttattttatctttttttttttttttttaagagatagggcatctaacggcattgttttagctgctcaacacttttttttttttgcttatttttgtttgttttgtttgtttttgagacagggtctccctctgttgcccagcatatagtgcagtggcatgatcatggctcactgcagcctcaacctcccaggatcaggcaatcctcctgcttcagcttcctgagtagctgagaccacaggtgcacaccaatatacctaatttttttttttttgagatggagtttcactcttgttgcccaggctggagtgcaatggcgtggtctcagctcactgcaacctctgcctccctggttcaagcgattctcctgtctcagcctgccgagtagctggggttacaggcataagccactacgcccagctaattttgtatttttagtagagacagggtttctccatgttggtcaggctggtctcgaactcctgacctcaggtgatccacccacctcagccttccaaagtgctgagattgcaggtgtgaaccactacgcctggccacctgactaatttttaagttattcacagagaacaggttttgcaatgttgcccaggctggtctcaaactcctgggctcaaatgatcctcctccctcggcctcccaaagtgctggggttacaggtgtgccactgtgcctggtcggctcaccactttcagatctggctctcttcacctctcttttatagtcataagctgattagcacaattctagacatccgcagctacatttaaggcaggaaggaggtggtaatagacactaccagccacatctgtcccttttaatcaggataccctagaaatcctcagcagactttgaattatgtgccattggtgaaatgtcatatgatcatccctctacaaggcaacgaggtaaaaagagaatttagtatttctagcctctagagtggagatgaacaaagaataggaatgggcatttgcttaggaaaccaactgtgccttacaacatttttgcacttttttctgtaacattttgtgttaaatcatataaaaatgctgatcctaacaaatatggtcaatgagtcacaccataattctctaagaactccagtccaaaaaggttaatcttgcttttaaactccaggcgcggtgtttcacagctgtaattttagcacttcgggaggcagagcaagaggatcacttgaggccaggagttggagaccagcctggcaacatagcaagaccccgtctctacaaaaaataaaattatctgggcctgttggtgcacacctgtagtcccagctactcaggaggctgaggtgggaggatcacttgagcctaggaattcgaggctgcagtgagctgtgattgcaccactgcactccagcctgggtgacagagggagaacctatctccaaaacaaaacaaaataaaaacaaaacaaaactccaagcagagaaagacttgacgagtcggatgagtctgatgattcctaaaggaaatcctttttgagattccaggagattccatctcctcaacagagtaattgattttgagcctcccacctcctgaattaaggcccacccatccctatcctgcactgaactgtagactcttttttacttccttacaaaagtttattcttaaatgtacaacagactccaagacgacactttattgtagctataggtggcaaaagatgttatggcagagaatccagatgtttaaataggaatggggtcaagggtcaccgccccaagcacggataacaaaatttattttttgccagatttctttaattccacctgtgactggtgagggctggtggcggggtggctttcacttttagctcctctttttgtttctgcttgaacgtcccatcttccttacccacccccttgacctgcttcttgagctttctcagggcttcttgccacctttgcagctgtacatggcacctgccatagggctctaattttaaactgagaaattgagaaaacaggaaactgactctttttggggggagagtaagacaaacaggaaaaggaaaatgaagacgtggttgatacagatcgttggatttcaaaaggaaaagtctacggataaccgaaaaaaataaatatttagaaatgcatagtcttggctggttaaataagtatccatgcttgttcttgtggcatagtagttacgagacatttttagttaaatggaaaaatgtgaattactatagtttgagtgatatgctgctttccaaattaaaagcagcataacaaaaacattcccctaatactcataaataattcattgaattggcaataattcacctcctaatgacttcatatgaagtataaagtaacttcgatacatcagaagaaatcctatcttctaatataagaaagtaatatgattacattaaatgcgtctcatataagttataaaaatggtatctatgagtaaagaaatgcttgtgaacaaaaaaattgatcttataaaggtcaaacaggccaggcgtggtggctcacacctgtaatcccagcactttgggaggctgaggtgggcggagtacctgaggtcaggagttcaagaccagcctggccaacatggtgataccctgtctctacaaaaatacaaaaaattagctgggcatgatggtgggtgcctgtaatctcagctactcgggaggcagaggcgggagaatcgcttgaacccgggaggcggaggttgcagtgaactgagattgagccacaacaaccaagcctgggagacagaggaaactctgtctcaaaaaataaaaaataaaaattaaaattaaaaaaaaggtcaaacaaaccaaacccttctgattaatttattcaatctacttttattataagcaaatgagaaattataattttaatctgaaaaagcagaatcaggggattttggagctggacagtcccctggaaattatttggatcaaagccctcattttataggtgaagaaactgagaagtaagatttgagcaagctgcccaaaggctttgccaaaggctataccagtgaatggcagagtctggactggaagtcccagtgctgccgtccaggtgagacctgttccactgcatgctactagctcccgggctgagaccggacttttgcttggcaggtttctttctttcgaaactattaattattgtattttttgtagagacagggttttgccatgatgcccaggctggtcttgaactcctgagctcaagagatccacccagcttggcctctcaaaaatgttgggattacaggcataagccacagtgcccggcccattttcctcccacctctttgttccttctctgtttcttttgcagcattatgttctatcattgtataccagagttcctcaacttcagttatagtctgttcttgctttatgctatcttcttcagcaagctcatcttggtctgttttcctccttatcaggcataccccagaaactcctgttttatctccacctcaactaaacattttcctgagttctgggcctctataaactaattatttgattaacatcttttttttttttttctgagatagagtctctctctgtcacccaggctggagtgcagtggtgcaatctcagatcactgcagcttctgcctcccagattcaagcgattctcctgcctcagcctcctaagtagctgggattataggcatgcaccaccgcacacagctaatttttgtacttttagtagagacggggtttcaccatgttggtcaggctggtctcaaactcctgatctgaagtgatctgactgcctcagcttcccaaagtgctgggattacaagcctgagccaccatgcctggccaacatctttaattggatatctcagtatcaagaaggcccataatattcctctgcctcatccctctcctcagtcctcttcttgtgtttcctagttcagagaatggcaccattctctatcaagctgcgcaaatcagacatgtgtgattttttgttgttgttgagacagggactcactctgtcacccaggctagagtgcagtggcgtgatcatggcgcactgaagcctcaaactcctgggctcaggagatcctcccgcctcagcctcctgagtagctgggaccacaggcccacaccaccatgcccagctaattttgtattctttgtagagatggggtttcatcatgtttgcccaggctggtctcgaactcctggactcaagcaatccacccacctcagcctcccaaagtgctgggattacaggcatgagccactgtgcccagctgaagtgtgatccttaacttcaccccttctcatgccctccatttccaatccatctccagtccagttgactccagctactcaattatttccacttatctcattccactacctttgaagctaccaccatctctaactacagtcatctcccaactaactggtctcctggcatctctctggttctcctccactaatttcaaaaaaagaaatttactgtgacagtgctcacaacactcccccttgctcttactaaagatgcttaccatagcctccaggtattgtatggcctgaggtctatctacatttccaggtgcaggacacaccatgtctccccactcccaaatttagtctccagactccatcctttttacagttctttaaaagcatcacaattcctccaaccactaggcatttgtatgtgctattccctctttccagaatgcaataccctccctctgcctagctagctaacttctatgtatctatgactgcagctcaaactttcctcatggactccctccacaagtgccaagcctgggccagattcttttgttatgtgctcacagaacgatgttccctttagcattcattgagtttgctgtttaattattcttgtcttgtttttgtttaattagtcctatctctaatactagacaaatgttccttaagatcacaggaaatataggactgtctctacataaaaactgttttatatccataatgcctaggacagtacctggcacacagtatatgctcaataaatttttgttgaatgaatgcaattatcattatattcctgatattagcaggtataatccagtttaagtttgggaacagaaagacaaaacggaccacatctaataaatccggtctcctttcttttattatttatttatttgagacagttttgctcttgttgcccaggctgcagtgcaatggcatgatcttggctcactgaaacctccgcctcccaagttcaagggattctccagcctcagcctcccaagtagctgggattacaggcatccaccaccacgcccagctaatttttttgtatttttagtagagatggggtttcaccatgttggccaggctggtctcgaactcctgacctcaggtgatccacccacctcagcctcccaaagtgttgggattacaggcgtgagccaccgtgcccggccaaggtctcctttcttttaatcaaactctcacctttggccattctgcagtcattcacccgacagtatttactgacggagtgaatacagagtgcttgattaatgttgctgctttgttattattattattattattgagatggagtcttgctctgttgcccaggctggagtgcagtggcgtgatctcggctcactgcaacctccgcctcccgggttcaagccattctcctgcctcagcctcccaagtagctgggactacaggcatgcaacaccacacctggctaatttttgtatttttagtagagacaaggtttcaccatattggccaggctggtcttgaactcctgacctcaggtgatctgcccacctcagcttcccaaagtgctgggattacaggcgtgagccaccatacccaacctaatgtttctgctttgaaatacaatttcaaaaagtcattaataggttgaaaacagcaagattttaaaagtattttaaaaagtgaaacagaagaatgcttacttcatttcacagagatagatttctcctttatgttatttctaaaaggagatggaattttgtttcattcatttctgcttatttggacaggccaaatatgaacagctgaacacgtcagcgttaccatgcatatgttacacagatgccatccttcttccatcagctctcatatgcaatacagaagtaaaaagaggttctctttatttttaaaaggtaaaaattgaaattcagtcacttaacacagaataaacaataattacaattacactggtaacaaaggacagcaagcatgttttctttgaaagcactgtatctggtttgtctccgtgcttggtcctagtatctggcatattttccccagagttttcttttcagtgggatgattatcttcggggcaaaaaagtttatcagactcaagttttagcagtacttattttattcatttatatacatgtaaccccatcctgtcttactccaatcttcttactgccttcctactgacacatatattatataacaccctccccaagttctatttacggttaaaaatttctttttttttttctttttttgagacagagtttcactctcgtcacccaggctggtgtgcaatggcgcagtctcggctcactgcaacctccgactccctggttcaagtgattctcctgtctcagcctcccgagtagctggaattacaggcgcccgccaccatgcccagctaatttttgtatttttagtagagacagtgtttcgccatgttggccaggctggtctcaaactcctgacctcaggtgatccacccgccttggcctctcaaagtgctgggattataggcgtaagccactgcgcccagcctacagttacgaatttctaaatggcacaaataaactcagctgttctcagtgcagacgtcaaatcctcactgtgctgaaacattttcctcagcttttgggaaataattacaatttaaacatacacagagaatgtttcttagacaaacataatacccgaggcttatctggtaaaaactaattgctctgtccttagcacaaaaaatatatatctttgtaaaatgagaagaaccaaagaatatttaaaacaaagaaggaagccacacgtactaattacacaagagactgactgacaaactggaattctccaaaacagattttcagcgaggcttctcatttcagagtccaggaaaaaaaaatcctaaaaaccccaaaggtatattatatgtgtgtatatatatttttattgtgttaaaaaacacaaaacataaaatttactgtcttatcaaaaggtatattttgtcgctcttccctttttttttttttttttttcccgagacagagtccagtctgtcgcccaggctgaagtgcagtggcatgatctcggctcactgcaacctgcatcttctgggctcaagcaatcctcccacctcagcctcctgagtagatggagctacaggcacgtgccactaggcccggctaatttttgtattttttgcagacagggttttgccatgttgcccgggctggtctttgttctcctaagagttgttttctccatgaaagttgataaataacatttagaaaatgaattattacaagagtaatgatatgtctcaatttattatatgaaattatcaacaactgcttttaatattcagatgtcaagaagatgaaaagcagaaatacattttgcaaacatgtagcactccataaatggaaatcatgtatttcctctaatatcccaatttttctatattgggatcttatatggctgtttctatatggctattttgtcccaacttgctgtacaagaattttccccagccaccttagaaaggttggatgtagttcactccaagtttgcagttcactccaagtgtttcagtaccacagaaagctccatggaagcctcaaatgtacgggctaggcaatagaagcagggaggtaggattaagaaattactggccaggtgtggtggctcaggcctgtaatcccagcacttcgagaggctgaggcagacagatggcttgagctcaagagtttgagatcagcctgagcaacatggcaaaactctgtctctacaaaaaatataaaaatcagccaggtatgttggtgtgcacctgtagtcccagctactggggaggttgaggcaggaggattgcttgagcccaggaggctgaggctgcagtgagccatgattgtgccactgcattccagcctggtcgactgtaagacaaaaaataagaaaataaaaaatttaccaatataaaatgctcaaacagctaacaaacatgttcaattccatttatagtcttttctttgagccatttaaacatagggctattttttttttttttttttgagatggagtttcactcttgttgcccaggctggagagcaatggcatgatctcggctcaccacaacctctgcctcctgggttcaagcgattctcctgcctcagcctcccgagcagctgggattacaggcatgtgccaccatgcctggctaattttgtatttttagtagagacgggattcctccatgttggtcagactggtcttgaactcccaacctcaggtgatctgcctgcctcaaccttccaaagtgctgggattacaggtgtgagccactgagattggctgccgttttgttttttaactccatatagtttctatagttcactgaaaactcaaagagatgacctataaatgtatgaataatgtatgatttcttacatcaattttctactagaaaaaaatcatacttttagaattggattttgtcttacagtcatctttattatactttataaatgagatttcatttatataaatcaggaagctaaactaaaatagaaacactagatttaaattctgatttgaatactctgatcaaaataacaaatctcacactgggaaaccatctatcagcaagcagagagctactgtgtgtccttccttagaagagtttgaacaccgagaacccacagcatatttgcagtacagtaacagcaattcctttgtcattatcacagaactttaattttcatatactttgctgggaccaaccaaaccatcccatatatataaccatatccatatatatatatatatatatcccacatatatatgggatggtatatatatacacatgtatatgtatgtgtgtgtgtatatatgtgtatatatgtatacacacacacacacacacatatatatatatatacacacacacacatatatatatggagagagagagagagacagtgtcttgctctgtcgcccaggctggagtgcagtggtacgatcttggctcattgcaacctccgcctcccaggctcaagcgattctcatgtctcagtctcccaagtagctgggattacaggtgtgcaccaccacaccaggctaaccattccatacattttatacaatcatttttaaaaagaagcatgaaccatttcggttttagagaattaagtttttttaaaaaagagactcttaaaaaaaagtcattatatgaataaaatctgctttgtgttaattccgacaaatcattccatcattgagtctgtcaccaattttttttttttgaaatggagtttcgctcttgttgcccaggctggagtgcaatggtacgatctcggctcactgcaaccgccgcctcccgggttcaagtgattctcctgcctcagcctcccgagtagctgggattacaggcatgcgccaccacgcctggctaattttgtattattagttgagacagggtttctccatgttggtcaggctggtctcgaactcctgacctcaagtgatccgctggccttggcctcccaaagtgctgggattacaggcgtgagccaccgtgcctggcccaattttttttttttaataacttgcacacttaacaatattttttatcttcttgggacaacattcttttctccacaaaaacccaattaaggacgttgtgccagtttactcctacttccttcctgttcactgagcttaaagtgggtataggcgagaatgccaaataatgtacataaaatgccaagggcctgattaatggacagtggatccttaaataaaacatatcctccgaataaagtaatgcagaacttgaagtgtccgaacatgttataggtgacaggtgaagtgttcccaatgatccaataaattgataagttcaccatgaaagctattactccagatagcagcaccataagcaaagcagaaactgaccagggaccaaatattcctccttctccaaacactggctcaaagaagggcacagcaaccagcaacatggcagatgacatcggagcctggtagtacagcagctgcattgagttcacttgtaattcatgctgtttggctcctacccaaaacaggtaggtatttggtgagcatcacacacccaagtttctctgtctcctttcttctcttcaccttgagtcagacaacttatgcaattatgctttcttcccaacagtctattgtctctatactgtattttctaaaccttggaatacagcttcaaaatttatgaaatctgcagcgtgagctggattctggtggagaaggttttctggtagcagaaggtctggatggctatgatcaccggcgtggtcatggccttggccagctgataggtgcctatggtgttgttctgcagagaaaggttagtgaagaccacaaagccacagaagctgagggccaggaggaggagcctggagggcggcagacttttgggggcaaagatgtccagcttctggcagatatacaagcccagccaggtgaccacgaagtgcaccagggtcaggctcatgttggggaagccgtggtacacataaatccatttgttgaggaacacaatgcagatggacaccagcaggttgaacaggagcccggcggcgattcgccagtggccccgcactcggtccaccagcaatgccatgatccccgcgaagctggggccgtctagcctcggaaggggcgccgggcctgtctccggctgcccttctactccaccgccgcgtcctcgcagacgccgacctcaccgtctgacccaggagtggcatgcacagatcaaccccgggcgagtagcactcttaacagaggacacacaccccgccgccgccctgtaagccagctaggac

SEQ ID NO: 11026 - RNA, 12834 nt, Homo sapiens
  source 1..12834: mol_type = other RNA
ctgaatagctgggactacaggtgcacaccatcacagctgactaatttttcttttctttttttttttttgagacggagtctcactctgtctcccaggctggagtgcagtgatgtgatctcagctcactgcaacctacgtctccagggttcatgtgagtttcctgcctcagcctcctgagtgagtagctgggattacaggcgcctgccaccacgtccagctaatttttgtatttttagtagagattgggtttcaccatgttggccaggctggtctccaactcctgacctcaagtgatccacctgcctcggcctcccaaatcgctgggattacaggcgtgagtcatcatgcctggccttttttttttttttgtgagacagagttttgctcttgtcacccaggctggagtgtaatggcatgatctcggctcactgaaacctctgccaggcacacgtcaccatgcccggctaatttttgtatttttggtagaaacggggtttcaccatgttggccaggctggtctccaactcctgacctcaagtgatcctcctgccttggcctcccaaagtgctgggattacaggtgttagctaccaagtctggcctttttttttttttttttttttttttttttttgagacagagtttcgctcttgtcacccaggctggagtgtaatagtgtgattccagcttactgcaacctctgcctctcgggttcaagccattctcctgcctcagcctcctgagcagctgggattacaggcacacgccagcatgcctggctaatttttatatttttagtagagacggggtttcaccatgttggccaggctggtctcgaactcctgacctcaggtgatccatctgcctcagcctcccaaactgctgggatgacaggcgtgagccaccacgccaggccctatttttatttttaaccagtgctgtagtttgaatatttgtctcctccaaaactcatctggaaacatccccaatgtggcaatattgagagatggcgcctttaaaaggtgactgggtcatgaaggctctgcccagtgagactggtgcctttataagaagaggaagagagacctgagctaccatgctcaagtccctcaccacgtgaggccctctgccaccttgggtctctgcagagagttcccaggaacaagaagtctctcaccagatgtggaccctgtaccttggacttctcagtctccactattgtaagaaataaattccttttctttataaatgacccagtttcaggtattctgttctatgcaacacaaaatggactaagacaacgagtacgcttagttgttgcttcctgagttccaaagtccgacagacagagcaggtcctccattcttgcccctttttaccccaaatgctcattggcattcttgcagctacgagtaataattaaaagtggctaagccaggctggcatggttgctcacgcctgtaatatcagcactttgggaggctgaggcaggaggatcacttgaacccaggagtgagaccagccagggcaacatagcaacaccctgtctctaattattattatttttttaagtgagtaagccaaataggggtttacttttcatctagaacaagaagacgtgttggccaggctggtctcaaactactgggctcaagtgatccacccacctcagcctcccaaagtgttgggattatgcgtgagccaccgcacctggccacaagacccaatttcttttattttatctttttttttttttttttaagagatagggcatctaacggcattgttttagctgctcaacacttttttttttttgcttatttttgtttgttttgtttgtttttgagacagggtctccctctgttgcccagcatatagtgcagtggcatgatcatggctcactgcagcctcaacctcccaggatcaggcaatcctcctgcttcagcttcctgagtagctgagaccacaggtgcacaccaatatacctaatttttttttttttgagatggagtttcactcttgttgcccaggctggagtgcaatggcgtggtctcagctcactgcaacctctgcctccctggttcaagcgattctcctgtctcagcctgccgagtagctggggttacaggcataagccactacgcccagctaattttgtatttttagtagagacagggtttctccatgttggtcaggctggtctcgaactcctgacctcaggtgatccacccacctcagccttccaaagtgctgagattgcaggtgtgaaccactacgcctggccacctgactaatttttaagttattcacagagaacaggttttgcaatgttgcccaggctggtctcaaactcctgggctcaaatgatcctcctccctcggcctcccaaagtgctggggttacaggtgtgccactgtgcctggtcggctcaccactttcagatctggctctcttcacctctcttttatagtcataagctgattagcacaattctagacatccgcagctacatttaaggcaggaaggaggtggtaatagacactaccagccacatctgtcccttttaatcaggataccctagaaatcctcagcagactttgaattatgtgccattggtgaaatgtcatatgatcatccctctacaaggcaacgaggtaaaaagagaatttagtatttctagcctctagagtggagatgaacaaagaataggaatgggcatttgcttaggaaaccaactgtgccttacaacatttttgcacttttttctgtaacattttgtgttaaatcatataaaaatgctgatcctaacaaatatggtcaatgagtcacaccataattctctaagaactccagtccaaaaaggttaatcttgcttttaaactccaggcgcggtgtttcacagctgtaattttagcacttcgggaggcagagcaagaggatcacttgaggccaggagttggagaccagcctggcaacatagcaagaccccgtctctacaaaaaataaaattatctgggcctgttggtgcacacctgtagtcccagctactcaggaggctgaggtgggaggatcacttgagcctaggaattcgaggctgcagtgagctgtgattgcaccactgcactccagcctgggtgacagagggagaacctatctccaaaacaaaacaaaataaaaacaaaacaaaactccaagcagagaaagacttgacgagtcggatgagtctgatgattcctaaaggaaatcctttttgagattccaggagattccatctcctcaacagagtaattgattttgagcctcccacctcctgaattaaggcccacccatccctatcctgcactgaactgtagactcttttttacttccttacaaaagtttattcttaaatgtacaacagactccaagacgacactttattgtagctataggtggcaaaagatgttatggcagagaatccagatgtttaaataggaatggggtcaagggtcaccgccccaagcacggataacaaaatttattttttgccagatttctttaattccacctgtgactggtgagggctggtggcggggtggctttcacttttagctcctctttttgtttctgcttgaacgtcccatcttccttacccacccccttgacctgcttcttgagctttctcagggcttcttgccacctttgcagctgtacatggcacctgccatagggctctaattttaaactgagaaattgagaaaacaggaaactgactctttttggggggagagtaagacaaacaggaaaaggaaaatgaagacgtggttgatacagatcgttggatttcaaaaggaaaagtctacggataaccgaaaaaaataaatatttagaaatgcatagtcttggctggttaaataagtatccatgcttgttcttgtggcatagtagttacgagacatttttagttaaatggaaaaatgtgaattactatagtttgagtgatatgctgctttccaaattaaaagcagcataacaaaaacattcccctaatactcataaataattcattgaattggcaataattcacctcctaatgacttcatatgaagtataaagtaacttcgatacatcagaagaaatcctatcttctaatataagaaagtaatatgattacattaaatgcgtctcatataagttataaaaatggtatctatgagtaaagaaatgcttgtgaacaaaaaaattgatcttataaaggtcaaacaggccaggcgtggtggctcacacctgtaatcccagcactttgggaggctgaggtgggcggagtacctgaggtcaggagttcaagaccagcctggccaacatggtgataccctgtctctacaaaaatacaaaaaattagctgggcatgatggtgggtgcctgtaatctcagctactcgggaggcagaggcgggagaatcgcttgaacccgggaggcggaggttgcagtgaactgagattgagccacaacaaccaagcctgggagacagaggaaactctgtctcaaaaaataaaaaataaaaattaaaattaaaaaaaaggtcaaacaaaccaaacccttctgattaatttattcaatctacttttattataagcaaatgagaaattataattttaatctgaaaaagcagaatcaggggattttggagctggacagtcccctggaaattatttggatcaaagccctcattttataggtgaagaaactgagaagtaagatttgagcaagctgcccaaaggctttgccaaaggctataccagtgaatggcagagtctggactggaagtcccagtgctgccgtccaggtgagacctgttccactgcatgctactagctcccgggctgagaccggacttttgcttggcaggtttctttctttcgaaactattaattattgtattttttgtagagacagggttttgccatgatgcccaggctggtcttgaactcctgagctcaagagatccacccagcttggcctctcaaaaatgttgggattacaggcataagccacagtgcccggcccattttcctcccacctctttgttccttctctgtttcttttgcagcattatgttctatcattgtataccagagttcctcaacttcagttatagtctgttcttgctttatgctatcttcttcagcaagctcatcttggtctgttttcctccttatcaggcataccccagaaactcctgttttatctccacctcaactaaacattttcctgagttctgggcctctataaactaattatttgattaacatcttttttttttttttctgagatagagtctctctctgtcacccaggctggagtgcagtggtgcaatctcagatcactgcagcttctgcctcccagattcaagcgattctcctgcctcagcctcctaagtagctgggattataggcatgcaccaccgcacacagctaatttttgtacttttagtagagacggggtttcaccatgttggtcaggctggtctcaaactcctgatctgaagtgatctgactgcctcagcttcccaaagtgctgggattacaagcctgagccaccatgcctggccaacatctttaattggatatctcagtatcaagaaggcccataatattcctctgcctcatccctctcctcagtcctcttcttgtgtttcctagttcagagaatggcaccattctctatcaagctgcgcaaatcagacatgtgtgattttttgttgttgttgagacagggactcactctgtcacccaggctagagtgcagtggcgtgatcatggcgcactgaagcctcaaactcctgggctcaggagatcctcccgcctcagcctcctgagtagctgggaccacaggcccacaccaccatgcccagctaattttgtattctttgtagagatggggtttcatcatgtttgcccaggctggtctcgaactcctggactcaagcaatccacccacctcagcctcccaaagtgctgggattacaggcatgagccactgtgcccagctgaagtgtgatccttaacttcaccccttctcatgccctccatttccaatccatctccagtccagttgactccagctactcaattatttccacttatctcattccactacctttgaagctaccaccatctctaactacagtcatctcccaactaactggtctcctggcatctctctggttctcctccactaatttcaaaaaaagaaatttactgtgacagtgctcacaacactcccccttgctcttactaaagatgcttaccatagcctccaggtattgtatggcctgaggtctatctacatttccaggtgcaggacacaccatgtctccccactcccaaatttagtctccagactccatcctttttacagttctttaaaagcatcacaattcctccaaccactaggcatttgtatgtgctattccctctttccagaatgcaataccctccctctgcctagctagctaacttctatgtatctatgactgcagctcaaactttcctcatggactccctccacaagtgccaagcctgggccagattcttttgttatgtgctcacagaacgatgttccctttagcattcattgagtttgctgtttaattattcttgtcttgtttttgtttaattagtcctatctctaatactagacaaatgttccttaagatcacaggaaatataggactgtctctacataaaaactgttttatatccataatgcctaggacagtacctggcacacagtatatgctcaataaatttttgttgaatgaatgcaattatcattatattcctgatattagcaggtataatccagtttaagtttgggaacagaaagacaaaacggaccacatctaataaatccggtctcctttcttttattatttatttatttgagacagttttgctcttgttgcccaggctgcagtgcaatggcatgatcttggctcactgaaacctccgcctcccaagttcaagggattctccagcctcagcctcccaagtagctgggattacaggcatccaccaccacgcccagctaatttttttgtatttttagtagagatggggtttcaccatgttggccaggctggtctcgaactcctgacctcaggtgatccacccacctcagcctcccaaagtgttgggattacaggcgtgagccaccgtgcccggccaaggtctcctttcttttaatcaaactctcacctttggccattctgcagtcattcacccgacagtatttactgacggagtgaatacagagtgcttgattaatgttgctgctttgttattattattattattattgagatggagtcttgctctgttgcccaggctggagtgcagtggcgtgatctcggctcactgcaacctccgcctcccgggttcaagccattctcctgcctcagcctcccaagtagctgggactacaggcatgcaacaccacacctggctaatttttgtatttttagtagagacaaggtttcaccatattggccaggctggtcttgaactcctgacctcaggtgatctgcccacctcagcttcccaaagtgctgggattacaggcgtgagccaccatacccaacctaatgtttctgctttgaaatacaatttcaaaaagtcattaataggttgaaaacagcaagattttaaaagtattttaaaaagtgaaacagaagaatgcttacttcatttcacagagatagatttctcctttatgttatttctaaaaggagatggaattttgtttcattcatttctgcttatttggacaggccaaatatgaacagctgaacacgtcagcgttaccatgcatatgttacacagatgccatccttcttccatcagctctcatatgcaatacagaagtaaaaagaggttctctttatttttaaaaggtaaaaattgaaattcagtcacttaacacagaataaacaataattacaattacactggtaacaaaggacagcaagcatgttttctttgaaagcactgtatctggtttgtctccgtgcttggtcctagtatctggcatattttccccagagttttcttttcagtgggatgattatcttcggggcaaaaaagtttatcagactcaagttttagcagtacttattttattcatttatatacatgtaaccccatcctgtcttactccaatcttcttactgccttcctactgacacatatattatataacaccctccccaagttctatttacggttaaaaatttctttttttttttctttttttgagacagagtttcactctcgtcacccaggctggtgtgcaatggcgcagtctcggctcactgcaacctccgactccctggttcaagtgattctcctgtctcagcctcccgagtagctggaattacaggcgcccgccaccatgcccagctaatttttgtatttttagtagagacagtgtttcgccatgttggccaggctggtctcaaactcctgacctcaggtgatccacccgccttggcctctcaaagtgctgggattataggcgtaagccactgcgcccagcctacagttacgaatttctaaatggcacaaataaactcagctgttctcagtgcagacgtcaaatcctcactgtgctgaaacattttcctcagcttttgggaaataattacaatttaaacatacacagagaatgtttcttagacaaacataatacccgaggcttatctggtaaaaactaattgctctgtccttagcacaaaaaatatatatctttgtaaaatgagaagaaccaaagaatatttaaaacaaagaaggaagccacacgtactaattacacaagagactgactgacaaactggaattctccaaaacagattttcagcgaggcttctcatttcagagtccaggaaaaaaaaatcctaaaaaccccaaaggtatattatatgtgtgtatatatatttttattgtgttaaaaaacacaaaacataaaatttactgtcttatcaaaaggtatattttgtcgctcttccctttttttttttttttttttcccgagacagagtccagtctgtcgcccaggctgaagtgcagtggcatgatctcggctcactgcaacctgcatcttctgggctcaagcaatcctcccacctcagcctcctgagtagatggagctacaggcacgtgccactaggcccggctaatttttgtattttttgcagacagggttttgccatgttgcccgggctggtctttgttctcctaagagttgttttctccatgaaagttgataaataacatttagaaaatgaattattacaagagtaatgatatgtctcaatttattatatgaaattatcaacaactgcttttaatattcagatgtcaagaagatgaaaagcagaaatacattttgcaaacatgtagcactccataaatggaaatcatgtatttcctctaatatcccaatttttctatattgggatcttatatggctgtttctatatggctattttgtcccaacttgctgtacaagaattttccccagccaccttagaaaggttggatgtagttcactccaagtttgcagttcactccaagtgtttcagtaccacagaaagctccatggaagcctcaaatgtacgggctaggcaatagaagcagggaggtaggattaagaaattactggccaggtgtggtggctcaggcctgtaatcccagcacttcgagaggctgaggcagacagatggcttgagctcaagagtttgagatcagcctgagcaacatggcaaaactctgtctctacaaaaaatataaaaatcagccaggtatgttggtgtgcacctgtagtcccagctactggggaggttgaggcaggaggattgcttgagcccaggaggctgaggctgcagtgagccatgattgtgccactgcattccagcctggtcgactgtaagacaaaaaataagaaaataaaaaatttaccaatataaaatgctcaaacagctaacaaacatgttcaattccatttatagtcttttctttgagccatttaaacatagggctattttttttttttttttttgagatggagtttcactcttgttgcccaggctggagagcaatggcatgatctcggctcaccacaacctctgcctcctgggttcaagcgattctcctgcctcagcctcccgagcagctgggattacaggcatgtgccaccatgcctggctaattttgtatttttagtagagacgggattcctccatgttggtcagactggtcttgaactcccaacctcaggtgatctgcctgcctcaaccttccaaagtgctgggattacaggtgtgagccactgagattggctgccgttttgttttttaactccatatagtttctatagttcactgaaaactcaaagagatgacctataaatgtatgaataatgtatgatttcttacatcaattttctactagaaaaaaatcatacttttagaattggattttgtcttacagtcatctttattatactttataaatgagatttcatttatataaatcaggaagctaaactaaaatagaaacactagatttaaattctgatttgaatactctgatcaaaataacaaatctcacactgggaaaccatctatcagcaagcagagagctactgtgtgtccttccttagaagagtttgaacaccgagaacccacagcatatttgcagtacagtaacagcaattcctttgtcattatcacagaactttaattttcatatactttgctgggaccaaccaaaccatcccatatatataaccatatccatatatatatatatatatatcccacatatatatgggatggtatatatatacacatgtatatgtatgtgtgtgtgtatatatgtgtatatatgtatacacacacacacacacacatatatatatatatacacacacacacatatatatatggagagagagagagagacagtgtcttgctctgtcgcccaggctggagtgcagtggtacgatcttggctcattgcaacctccgcctcccaggctcaagcgattctcatgtctcagtctcccaagtagctgggattacaggtgtgcaccaccacaccaggctaaccattccatacattttatacaatcatttttaaaaagaagcatgaaccatttcggttttagagaattaagtttttttaaaaaagagactcttaaaaaaaagtcattatatgaataaaatctgctttgtgttaattccgacaaatcattccatcattgagtctgtcaccaattttttttttttgaaatggagtttcgctcttgttgcccaggctggagtgcaatggtacgatctcggctcactgcaaccgccgcctcccgggttcaagtgattctcctgcctcagcctcccgagtagctgggattacaggcatgcgccaccacgcctggctaattttgtattattagttgagacagggtttctccatgttggtcaggctggtctcgaactcctgacctcaagtgatccgctggccttggcctcccaaagtgctgggattacaggcgtgagccaccgtgcctggcccaattttttttttttaataacttgcacacttaacaatattttttatcttcttgggacaacattcttttctccacaaaaacccaattaaggacgttgtgccagtttactcctacttccttcctgttcactgagcttaaagtgggtataggcgagaatgccaaataatgtacataaaatgccaagggcctgattaatggacagtggatccttaaataaaacatatcctccgaataaagtaatgcagaacttgaagtgtccgaacatgttataggtgacaggtgaagtgttcccaatgatccaataaattgataagttcaccatgaaagctattactccagatagcagcaccataagcaaagcagaaactgaccagggaccaaatattcctccttctccaaacactggctcaaagaagggcacagcaaccagcaacatggcagatgacatcggagcctggtagtacagcagctgcattgagttcacttgtaattcatgctgtttggctcctacccacacttgataaagggatgtaactaaaacaccaagagcagcaaacaccattccaaggaaattaaacttcacatcgtaataagaatttaggattacacctaaagttataggaatcagcgtgagctggattctggtggagaaggttttctggtagcagaaggtctggatggctatgatcaccggcgtggtcatggccttggccagctgataggtgcctatggtgttgttctgcagagaaaggttagtgaagaccacaaagccacagaagctgagggccaggaggaggagcctggagggcggcagacttttgggggcaaagatgtccagcttctggcagatatacaagcccagccaggtgaccacgaagtgcaccagggtcaggctcatgttggggaagccgtggtacacataaatccatttgttgaggaacacaatgcagatggacaccagcaggttgaacaggagcccggcggcgattcgccagtggccccgcactcggtccaccagcaatgccatgatccccgcgaagctggggccgtctagcctcggaaggggcgccgggcctgtctccggctgcccttctactccaccgccgcgtcctcgcagacgccgacctcaccgtctgacccaggagtggcatgcacagatcaaccccgggcgagtagcactcttaacagaggacacacaccccgccgccgccctgtaagccagctaggac

SEQ ID NO: 11027 - RNA, 12723 nt, Homo sapiens
  source 1..12723: mol_type = other RNA
ctgaatagctgggactacaggtgcacaccatcacagctgactaatttttcttttctttttttttttttgagacggagtctcactctgtctcccaggctggagtgcagtgatgtgatctcagctcactgcaacctacgtctccagggttcatgtgagtttcctgcctcagcctcctgagtgagtagctgggattacaggcgcctgccaccacgtccagctaatttttgtatttttagtagagattgggtttcaccatgttggccaggctggtctccaactcctgacctcaagtgatccacctgcctcggcctcccaaatcgctgggattacaggcgtgagtcatcatgcctggccttttttttttttttgtgagacagagttttgctcttgtcacccaggctggagtgtaatggcatgatctcggctcactgaaacctctgccaggcacacgtcaccatgcccggctaatttttgtatttttggtagaaacggggtttcaccatgttggccaggctggtctccaactcctgacctcaagtgatcctcctgccttggcctcccaaagtgctgggattacaggtgttagctaccaagtctggcctttttttttttttttttttttttttttttttgagacagagtttcgctcttgtcacccaggctggagtgtaatagtgtgattccagcttactgcaacctctgcctctcgggttcaagccattctcctgcctcagcctcctgagcagctgggattacaggcacacgccagcatgcctggctaatttttatatttttagtagagacggggtttcaccatgttggccaggctggtctcgaactcctgacctcaggtgatccatctgcctcagcctcccaaactgctgggatgacaggcgtgagccaccacgccaggccctatttttatttttaaccagtgctgtagtttgaatatttgtctcctccaaaactcatctggaaacatccccaatgtggcaatattgagagatggcgcctttaaaaggtgactgggtcatgaaggctctgcccagtgagactggtgcctttataagaagaggaagagagacctgagctaccatgctcaagtccctcaccacgtgaggccctctgccaccttgggtctctgcagagagttcccaggaacaagaagtctctcaccagatgtggaccctgtaccttggacttctcagtctccactattgtaagaaataaattccttttctttataaatgacccagtttcaggtattctgttctatgcaacacaaaatggactaagacaacgagtacgcttagttgttgcttcctgagttccaaagtccgacagacagagcaggtcctccattcttgcccctttttaccccaaatgctcattggcattcttgcagctacgagtaataattaaaagtggctaagccaggctggcatggttgctcacgcctgtaatatcagcactttgggaggctgaggcaggaggatcacttgaacccaggagtgagaccagccagggcaacatagcaacaccctgtctctaattattattatttttttaagtgagtaagccaaataggggtttacttttcatctagaacaagaagacgtgttggccaggctggtctcaaactactgggctcaagtgatccacccacctcagcctcccaaagtgttgggattatgcgtgagccaccgcacctggccacaagacccaatttcttttattttatctttttttttttttttttaagagatagggcatctaacggcattgttttagctgctcaacacttttttttttttgcttatttttgtttgttttgtttgtttttgagacagggtctccctctgttgcccagcatatagtgcagtggcatgatcatggctcactgcagcctcaacctcccaggatcaggcaatcctcctgcttcagcttcctgagtagctgagaccacaggtgcacaccaatatacctaatttttttttttttgagatggagtttcactcttgttgcccaggctggagtgcaatggcgtggtctcagctcactgcaacctctgcctccctggttcaagcgattctcctgtctcagcctgccgagtagctggggttacaggcataagccactacgcccagctaattttgtatttttagtagagacagggtttctccatgttggtcaggctggtctcgaactcctgacctcaggtgatccacccacctcagccttccaaagtgctgagattgcaggtgtgaaccactacgcctggccacctgactaatttttaagttattcacagagaacaggttttgcaatgttgcccaggctggtctcaaactcctgggctcaaatgatcctcctccctcggcctcccaaagtgctggggttacaggtgtgccactgtgcctggtcggctcaccactttcagatctggctctcttcacctctcttttatagtcataagctgattagcacaattctagacatccgcagctacatttaaggcaggaaggaggtggtaatagacactaccagccacatctgtcccttttaatcaggataccctagaaatcctcagcagactttgaattatgtgccattggtgaaatgtcatatgatcatccctctacaaggcaacgaggtaaaaagagaatttagtatttctagcctctagagtggagatgaacaaagaataggaatgggcatttgcttaggaaaccaactgtgccttacaacatttttgcacttttttctgtaacattttgtgttaaatcatataaaaatgctgatcctaacaaatatggtcaatgagtcacaccataattctctaagaactccagtccaaaaaggttaatcttgcttttaaactccaggcgcggtgtttcacagctgtaattttagcacttcgggaggcagagcaagaggatcacttgaggccaggagttggagaccagcctggcaacatagcaagaccccgtctctacaaaaaataaaattatctgggcctgttggtgcacacctgtagtcccagctactcaggaggctgaggtgggaggatcacttgagcctaggaattcgaggctgcagtgagctgtgattgcaccactgcactccagcctgggtgacagagggagaacctatctccaaaacaaaacaaaataaaaacaaaacaaaactccaagcagagaaagacttgacgagtcggatgagtctgatgattcctaaaggaaatcctttttgagattccaggagattccatctcctcaacagagtaattgattttgagcctcccacctcctgaattaaggcccacccatccctatcctgcactgaactgtagactcttttttacttccttacaaaagtttattcttaaatgtacaacagactccaagacgacactttattgtagctataggtggcaaaagatgttatggcagagaatccagatgtttaaataggaatggggtcaagggtcaccgccccaagcacggataacaaaatttattttttgccagatttctttaattccacctgtgactggtgagggctggtggcggggtggctttcacttttagctcctctttttgtttctgcttgaacgtcccatcttccttacccacccccttgacctgcttcttgagctttctcagggcttcttgccacctttgcagctgtacatggcacctgccatagggctctaattttaaactgagaaattgagaaaacaggaaactgactctttttggggggagagtaagacaaacaggaaaaggaaaatgaagacgtggttgatacagatcgttggatttcaaaaggaaaagtctacggataaccgaaaaaaataaatatttagaaatgcatagtcttggctggttaaataagtatccatgcttgttcttgtggcatagtagttacgagacatttttagttaaatggaaaaatgtgaattactatagtttgagtgatatgctgctttccaaattaaaagcagcataacaaaaacattcccctaatactcataaataattcattgaattggcaataattcacctcctaatgacttcatatgaagtataaagtaacttcgatacatcagaagaaatcctatcttctaatataagaaagtaatatgattacattaaatgcgtctcatataagttataaaaatggtatctatgagtaaagaaatgcttgtgaacaaaaaaattgatcttataaaggtcaaacaggccaggcgtggtggctcacacctgtaatcccagcactttgggaggctgaggtgggcggagtacctgaggtcaggagttcaagaccagcctggccaacatggtgataccctgtctctacaaaaatacaaaaaattagctgggcatgatggtgggtgcctgtaatctcagctactcgggaggcagaggcgggagaatcgcttgaacccgggaggcggaggttgcagtgaactgagattgagccacaacaaccaagcctgggagacagaggaaactctgtctcaaaaaataaaaaataaaaattaaaattaaaaaaaaggtcaaacaaaccaaacccttctgattaatttattcaatctacttttattataagcaaatgagaaattataattttaatctgaaaaagcagaatcaggggattttggagctggacagtcccctggaaattatttggatcaaagccctcattttataggtgaagaaactgagaagtaagatttgagcaagctgcccaaaggctttgccaaaggctataccagtgaatggcagagtctggactggaagtcccagtgctgccgtccaggtgagacctgttccactgcatgctactagctcccgggctgagaccggacttttgcttggcaggtttctttctttcgaaactattaattattgtattttttgtagagacagggttttgccatgatgcccaggctggtcttgaactcctgagctcaagagatccacccagcttggcctctcaaaaatgttgggattacaggcataagccacagtgcccggcccattttcctcccacctctttgttccttctctgtttcttttgcagcattatgttctatcattgtataccagagttcctcaacttcagttatagtctgttcttgctttatgctatcttcttcagcaagctcatcttggtctgttttcctccttatcaggcataccccagaaactcctgttttatctccacctcaactaaacattttcctgagttctgggcctctataaactaattatttgattaacatcttttttttttttttctgagatagagtctctctctgtcacccaggctggagtgcagtggtgcaatctcagatcactgcagcttctgcctcccagattcaagcgattctcctgcctcagcctcctaagtagctgggattataggcatgcaccaccgcacacagctaatttttgtacttttagtagagacggggtttcaccatgttggtcaggctggtctcaaactcctgatctgaagtgatctgactgcctcagcttcccaaagtgctgggattacaagcctgagccaccatgcctggccaacatctttaattggatatctcagtatcaagaaggcccataatattcctctgcctcatccctctcctcagtcctcttcttgtgtttcctagttcagagaatggcaccattctctatcaagctgcgcaaatcagacatgtgtgattttttgttgttgttgagacagggactcactctgtcacccaggctagagtgcagtggcgtgatcatggcgcactgaagcctcaaactcctgggctcaggagatcctcccgcctcagcctcctgagtagctgggaccacaggcccacaccaccatgcccagctaattttgtattctttgtagagatggggtttcatcatgtttgcccaggctggtctcgaactcctggactcaagcaatccacccacctcagcctcccaaagtgctgggattacaggcatgagccactgtgcccagctgaagtgtgatccttaacttcaccccttctcatgccctccatttccaatccatctccagtccagttgactccagctactcaattatttccacttatctcattccactacctttgaagctaccaccatctctaactacagtcatctcccaactaactggtctcctggcatctctctggttctcctccactaatttcaaaaaaagaaatttactgtgacagtgctcacaacactcccccttgctcttactaaagatgcttaccatagcctccaggtattgtatggcctgaggtctatctacatttccaggtgcaggacacaccatgtctccccactcccaaatttagtctccagactccatcctttttacagttctttaaaagcatcacaattcctccaaccactaggcatttgtatgtgctattccctctttccagaatgcaataccctccctctgcctagctagctaacttctatgtatctatgactgcagctcaaactttcctcatggactccctccacaagtgccaagcctgggccagattcttttgttatgtgctcacagaacgatgttccctttagcattcattgagtttgctgtttaattattcttgtcttgtttttgtttaattagtcctatctctaatactagacaaatgttccttaagatcacaggaaatataggactgtctctacataaaaactgttttatatccataatgcctaggacagtacctggcacacagtatatgctcaataaatttttgttgaatgaatgcaattatcattatattcctgatattagcaggtataatccagtttaagtttgggaacagaaagacaaaacggaccacatctaataaatccggtctcctttcttttattatttatttatttgagacagttttgctcttgttgcccaggctgcagtgcaatggcatgatcttggctcactgaaacctccgcctcccaagttcaagggattctccagcctcagcctcccaagtagctgggattacaggcatccaccaccacgcccagctaatttttttgtatttttagtagagatggggtttcaccatgttggccaggctggtctcgaactcctgacctcaggtgatccacccacctcagcctcccaaagtgttgggattacaggcgtgagccaccgtgcccggccaaggtctcctttcttttaatcaaactctcacctttggccattctgcagtcattcacccgacagtatttactgacggagtgaatacagagtgcttgattaatgttgctgctttgttattattattattattattgagatggagtcttgctctgttgcccaggctggagtgcagtggcgtgatctcggctcactgcaacctccgcctcccgggttcaagccattctcctgcctcagcctcccaagtagctgggactacaggcatgcaacaccacacctggctaatttttgtatttttagtagagacaaggtttcaccatattggccaggctggtcttgaactcctgacctcaggtgatctgcccacctcagcttcccaaagtgctgggattacaggcgtgagccaccatacccaacctaatgtttctgctttgaaatacaatttcaaaaagtcattaataggttgaaaacagcaagattttaaaagtattttaaaaagtgaaacagaagaatgcttacttcatttcacagagatagatttctcctttatgttatttctaaaaggagatggaattttgtttcattcatttctgcttatttggacaggccaaatatgaacagctgaacacgtcagcgttaccatgcatatgttacacagatgccatccttcttccatcagctctcatatgcaatacagaagtaaaaagaggttctctttatttttaaaaggtaaaaattgaaattcagtcacttaacacagaataaacaataattacaattacactggtaacaaaggacagcaagcatgttttctttgaaagcactgtatctggtttgtctccgtgcttggtcctagtatctggcatattttccccagagttttcttttcagtgggatgattatcttcggggcaaaaaagtttatcagactcaagttttagcagtacttattttattcatttatatacatgtaaccccatcctgtcttactccaatcttcttactgccttcctactgacacatatattatataacaccctccccaagttctatttacggttaaaaatttctttttttttttctttttttgagacagagtttcactctcgtcacccaggctggtgtgcaatggcgcagtctcggctcactgcaacctccgactccctggttcaagtgattctcctgtctcagcctcccgagtagctggaattacaggcgcccgccaccatgcccagctaatttttgtatttttagtagagacagtgtttcgccatgttggccaggctggtctcaaactcctgacctcaggtgatccacccgccttggcctctcaaagtgctgggattataggcgtaagccactgcgcccagcctacagttacgaatttctaaatggcacaaataaactcagctgttctcagtgcagacgtcaaatcctcactgtgctgaaacattttcctcagcttttgggaaataattacaatttaaacatacacagagaatgtttcttagacaaacataatacccgaggcttatctggtaaaaactaattgctctgtccttagcacaaaaaatatatatctttgtaaaatgagaagaaccaaagaatatttaaaacaaagaaggaagccacacgtactaattacacaagagactgactgacaaactggaattctccaaaacagattttcagcgaggcttctcatttcagagtccaggaaaaaaaaatcctaaaaaccccaaaggtatattatatgtgtgtatatatatttttattgtgttaaaaaacacaaaacataaaatttactgtcttatcaaaaggtatattttgtcgctcttccctttttttttttttttttttcccgagacagagtccagtctgtcgcccaggctgaagtgcagtggcatgatctcggctcactgcaacctgcatcttctgggctcaagcaatcctcccacctcagcctcctgagtagatggagctacaggcacgtgccactaggcccggctaatttttgtattttttgcagacagggttttgccatgttgcccgggctggtctttgttctcctaagagttgttttctccatgaaagttgataaataacatttagaaaatgaattattacaagagtaatgatatgtctcaatttattatatgaaattatcaacaactgcttttaatattcagatgtcaagaagatgaaaagcagaaatacattttgcaaacatgtagcactccataaatggaaatcatgtatttcctctaatatcccaatttttctatattgggatcttatatggctgtttctatatggctattttgtcccaacttgctgtacaagaattttccccagccaccttagaaaggttggatgtagttcactccaagtttgcagttcactccaagtgtttcagtaccacagaaagctccatggaagcctcaaatgtacgggctaggcaatagaagcagggaggtaggattaagaaattactggccaggtgtggtggctcaggcctgtaatcccagcacttcgagaggctgaggcagacagatggcttgagctcaagagtttgagatcagcctgagcaacatggcaaaactctgtctctacaaaaaatataaaaatcagccaggtatgttggtgtgcacctgtagtcccagctactggggaggttgaggcaggaggattgcttgagcccaggaggctgaggctgcagtgagccatgattgtgccactgcattccagcctggtcgactgtaagacaaaaaataagaaaataaaaaatttaccaatataaaatgctcaaacagctaacaaacatgttcaattccatttatagtcttttctttgagccatttaaacatagggctattttttttttttttttttgagatggagtttcactcttgttgcccaggctggagagcaatggcatgatctcggctcaccacaacctctgcctcctgggttcaagcgattctcctgcctcagcctcccgagcagctgggattacaggcatgtgccaccatgcctggctaattttgtatttttagtagagacgggattcctccatgttggtcagactggtcttgaactcccaacctcaggtgatctgcctgcctcaaccttccaaagtgctgggattacaggtgtgagccactgagattggctgccgttttgttttttaactccatatagtttctatagttcactgaaaactcaaagagatgacctataaatgtatgaataatgtatgatttcttacatcaattttctactagaaaaaaatcatacttttagaattggattttgtcttacagtcatctttattatactttataaatgagatttcatttatataaatcaggaagctaaactaaaatagaaacactagatttaaattctgatttgaatactctgatcaaaataacaaatctcacactgggaaaccatctatcagcaagcagagagctactgtgtgtccttccttagaagagtttgaacaccgagaacccacagcatatttgcagtacagtaacagcaattcctttgtcattatcacagaactttaattttcatatactttgctgggaccaaccaaaccatcccatatatataaccatatccatatatatatatatatatatcccacatatatatgggatggtatatatatacacatgtatatgtatgtgtgtgtgtatatatgtgtatatatgtatacacacacacacacacacatatatatatatatacacacacacacatatatatatggagagagagagagagacagtgtcttgctctgtcgcccaggctggagtgcagtggtacgatcttggctcattgcaacctccgcctcccaggctcaagcgattctcatgtctcagtctcccaagtagctgggattacaggtgtgcaccaccacaccaggctaaccattccatacattttatacaatcatttttaaaaagaagcatgaaccatttcggttttagagaattaagtttttttaaaaaagagactcttaaaaaaaagtcattatatgaataaaatctgctttgtgttaattccgacaaatcattccatcattgagtctgtcaccaattttttttttttgaaatggagtttcgctcttgttgcccaggctggagtgcaatggtacgatctcggctcactgcaaccgccgcctcccgggttcaagtgattctcctgcctcagcctcccgagtagctgggattacaggcatgcgccaccacgcctggctaattttgtattattagttgagacagggtttctccatgttggtcaggctggtctcgaactcctgacctcaagtgatccgctggccttggcctcccaaagtgctgggattacaggcgtgagccaccgtgcctggcccaattttttttttttaataacttgcacacttaacaatattttttatcttcttgggacaacattcttttctccacaaaaacccaattaaggacgttgtgccagtttactcctacttccttcctgttcactgagcttaaagtgggtataggcgagaatgccaaataatgtacataaaatgccaagggcctgattaatggacagtggatccttaaataaaacatatcctccgaataaagtaatgcagaacttgaagtgtccgaacatgttataggtgacaggtgaagtgttcccaatgatccaataaattgataagttcaccatgaaagctattactccagatagcagcaccataagcaaagcagaaactgaccagggaccaaatattcctccttctccaaacactggctcaaagaagggcacagcaaccagcaacatggcagatgacatcggagcctggtagtacagcagctgcattgagttcacttgtaattcatgctgtttggctcctacccacagcgtgagctggattctggtggagaaggttttctggtagcagaaggtctggatggctatgatcaccggcgtggtcatggccttggccagctgataggtgcctatggtgttgttctgcagagaaaggttagtgaagaccacaaagccacagaagctgagggccaggaggaggagcctggagggcggcagacttttgggggcaaagatgtccagcttctggcagatatacaagcccagccaggtgaccacgaagtgcaccagggtcaggctcatgttggggaagccgtggtacacataaatccatttgttgaggaacacaatgcagatggacaccagcaggttgaacaggagcccggcggcgattcgccagtggccccgcactcggtccaccagcaatgccatgatccccgcgaagctggggccgtctagcctcggaaggggcgccgggcctgtctccggctgcccttctactccaccgccgcgtcctcgcagacgccgacctcaccgtctgacccaggagtggcatgcacagatcaaccccgggcgagtagcactcttaacagaggacacacaccccgccgccgccctgtaagccagctaggac

SEQ ID NO: 11028 - RNA, 3724 nt, Homo sapiens
  source 1..3724: mol_type = other RNA
ctgaatagctgggactacaggtgcacaccatcacgcctggctattgtttttttgtttgtttttgtttttgtttgagatgaggtctcgctatgttgcccagtctgctctccaactcttggcctccagtgatcctcctgcttcggcttcccaaagcactgggattataggcatgagccaccatgcccggcagtgaagtattttctatccttgaaatgtgttagacaaattcctgaggggaaaccccacacattcaataacactttactttttcagcaaagcttcccatgtattggagcctcattttatccctcacccatgaactttaaaagtggaaaatcattttgttcttaaaaagaggaacagtcaggaaaaggtagggctctcaaatgatagtgagagctcagggactcgaacacttgatgcaacttgtcgagctcaggcccagccccgcgaggagctgagtcggggctggcgtgctggcgggacggtcagagctgcagccactgaggtcacgactacggaaaagcatcttctcttgagccgtgggggaaggtggggcgctggggcgcaggggcgcagcgggcgctggggacacacctgctggaactgcgcgcgggatccgcctcaccccaccttactccgccttctcctccctttcctccggcatcttcaccgacaggatctgctctcccggctccgggcccgggctcatgcagatcctcaccgagtgctcttcgggctcggccggcccctcctcctctccctccggcctcccaagggaggcaggcggtggagagctcggtggagaccccgggggctcggggggcgtccggggcgcgggtgggtcggtggcggcctcctttgggtgcgtgtgctggtctggggcggcggagccttcctctcccttgacgtcttgcgagctcttggcctgttccaccaactcttgctgctttgcagccgcctccagcgcggccagttctttgagccgggcccggaggtgagcaagtttgccgccttttgcccccttgccacccatctttcctgtcatagcgagggcagcgttgaagagctttggggtgcccgcccggggtggaaggatcagcacgctcttctcctccttgggcttattgttgcttctcagcatgcgcctggctttcttccggagtaacttctgagactcaggataatgcaccaaaatctcattcaggtccttcttatccaggatgaagaggttggtaaacccgtgcgccaccacgttggccgtgcgccggttcccgcccccaacagccagcaagcttatttctccaaacacagatccagctttcagcgtcaccagcacagatttcccatcagggccgcccaagacctgcacttgccctgcctggatgatgtacatctcacggccgatctcccccttcttgcacacatagtcgttgggcaggtagacaacagagcgaagcctcttcagcatgtcaaagatcatctgccggtcacagccctgaaagagtgcgactttgctaacgatgttgtagttcacgtcgatggcgaggtccagccgcatcttgtctggaagctgcaccatcagctctgactcatccagcatgccttgcgagtgccaggtgtactcgtaccaggtcttgacgcggttctgcacggacttggggatcttgtagaaattcatgtacttcaccgtgctgtccatgcagctgcggtagtaggtctgtccggcggtggcggcccctaccacatctctcatctgtccgatcatcacagagaaagcaaagacgcccgtgaaataattcagcagctggaagacaatttcaaagagtgtcttggggtcaggcagccccccgatggtgatgagggtcttcacagcaaagtagtaacagcgaatataactgtttcccacgccatcgtaaacccagtgagtggagccgaggccctgataggccgatgcccagtaataaagacaggaattcaaatgcaggctgtagagaaggtaggctgtggtcctgatgaccctgtacacgtaggctttgctgaggatggattccaggcggctgttaaactcgaagaaggccatgtactttaaacagcggggcaggcggaggagggggttcacaccgactttcaaatagagaaaatccaagggcaggaggctgagcaggtccatcttgaagcggcgagacttcaggtagttatttcgcatgtcctttttgtccgtaatgatgtccccgcctctgacaaactgcaggcgtgtctggaacacggtgatgtccaggaagtagatgaggtcgcataggtaatccatcagcagccagtggtggatgttgtccggggtctggtaggggaaggcccagcgcacgggaatcagccaacagttccaattccaggccatcaccacgaagaacagccataggacatacatcaggttggtcagcgggtcaatgctctggggaaactggtacttcttccaggggcggtgtttgaacttgcagcagagcatgtcgcaatagtgctcctcttccactggctcggcttcagcgggctttgtgtctggagctggctctggggctttcttggctggggagggcttggggctctcctcatcagaggtgacgtcagggtcaatgagtttctccttcactttctctgtccgctccttgaagagcttcaccagctcctggagccggtcgttgatgatggcgctatttgtgctggccgtggaggccgcacggtcctggccatcagtgtccttcggggtggtggggtcagaccaggcaaccactggggactctgctggtgacaacgccttgagctcttcagcctcatcatcctcagagggcagcttcttcctgtgtgtccccgaggctgagcttgggactataagggtgtctgatttggcaggagacggtggcggcaacacggttgagggtggattctcttctgccatgagggggcagctatcagcatcagtatcttccacctgcacttctgggtgctgtttcgtggcaggcactagttggcggatggagctcctggtctccttggcgaagctggagttggacaagctggttctccgggaggtgaggacagggatgcgggtgattgggatgcggtagctgggcacattagggagatgctctaccaggttttggagggcagaggcagaggccacctggccaggtatctggtcctggactaggcaattcagctccatgttctgacatggtgtagccatggtgctggggccagagagtctcaggcagaggagtgaccctggggactcctgaactggcagcctcggcctcagcctcaggctcctccttggtctccgcccagtcctggggctccttttcagcctcctcttcagccacctcctcggcctcctccttggccttctcttcagcctccttcttggcctcctccccaacttcctcccacagcttctgatctgaagtgctctggggccgggtcccgtcttcttcactctggcccacgcccacctgcgacaccacacagctatccagcagcaccttggatctctcggtcgggaccagtcaggatgcccatggtgcaggggttcagctgggggctgtggcgttcatcccaagcctgggtcggtgcatgcaagtgggagcccagctcccgagccagggtggctccagtggcagaggagccagcaatccttcctgcttctaatcagattgaggagatgtgcagg

SEQ ID NO: 11029 - RNA, 4467 nt, Homo sapiens
  source 1..4467: mol_type = other RNA
ctgaatagctgggactacaggtgcacaccatcacgcctggctattgtttttttgtttgtttttgtttttgtttgagatgaggtctcgctatgttgcccagtctgctctccaactcttggcctccagtgatcctcctgcttcggcttcccaaagcactgggattataggcatgagccaccatgcccggcagtgaagtattttctatccttgaaatgtgttagacaaattcctgaggggaaaccccacacattcaataacactttactttttcagcaaagcttcccatgtattggagcctcattttatccctcacccatgaactttaaaagtggaaaatcattttgttcttaaaaagaggaacagtcaggaaaaggtagggctctcaaatgatagtgagagctcagggactcgaacacttgatgcaacttgtcgagctcaggcccagccccgcgaggagctgagtcggggctggcgtgctggcgggacggtcagagctgcagccactgaggtcacgactacggaaaagcatcttctcttgagccgtgggggaaggtggggcgctggggcgcaggggcgcagcgggcgctggggacacacctgctggaactgcgcgcgggatccgcctcaccccaccttactccgccttctcctccctttcctccggcatcttcaccgacaggatctgctctcccggctccgggcccgggctcatgcagatcctcaccgagtgctcttcgggctcggccggcccctcctcctctccctccggcctcccaagggaggcaggcggtggagagctcggtggagaccccgggggctcggggggcgtccggggcgcgggtgggtcggtggcggcctcctttgggtgcgtgtgctggtctggggcggcggagccttcctctcccttgacgtcttgcgagctcttggcctgttccaccaactcttgctgctttgcagccgcctccagcgcggccagttctttgagccgggcccggaggtgagcaagtttgccgccttttgcccccttgccacccatctttcctgtcatagcgagggcagcgttgaagagctttggggtgcccgcccggggtggaaggatcagcacgctcttctcctccttgggcttattgttgcttctcagcatgcgcctggctttcttccggagtaacttctgagactcaggataatgcaccaaaatctcattcaggtccttcttatccaggatgaagaggttggtaaacccgtgcgccaccacgttggccgtgcgccggttcccgcccccaacagccagcaagcttatttctccaaacacagatccagctttcagcgtcaccagcacagatttcccatcagggccgcccaagacctgcacttgccctgcctggatgatgtacatctcacggccgatctcccccttcttgcacacatagtcgttgggcaggtagacaacagagcgaagcctcttcagcatgtcaaagatcatctgccggtcacagccctgaaagagtgcgactttgctaacgatgttgtagttcacgtcgatggcgaggtccagccgcatcttgtctggaagctgcaccatcagctctgactcatccagcatgccttgcgagtgccaggtgtactcgtaccaggtcttgacgcggttctgcacggacttggggatcttgtagaaattcatgtacttcaccgtgctgtccatgcagctgcggtagtaggtctgtccggcggtggcggcccctaccacatctctcatctgtccgatcatcacagagaaagcaaagacgcccgtgaaataattcagcagctggaagacaatttcaaagagtgtcttggggtcaggcagccccccgatggtgatgagggtcttcacagcaaagtagtaacagcgaatataactgtttcccacgccatcgtaaacccagtgagtggagccgaggccctgataggccgatgcccagtaataaagacaggaattcaaatgcaggctgtagagaaggtaggctgtggtcctgatgaccctgtacacgtaggctttgctgaggatggattccaggcggctgttaaactcgaagaaggccatgtactttaaacagcggggcaggcggaggagggggttcacaccgactttcaaatagagaaaatccaagggcaggaggctgagcaggtccatcttgaagcggcgagacttcaggtagttatttcgcatgtcctttttgtccgtaatgatgtccccgcctctgacaaactgcaggcgtgtctggaacacggtgatgtccaggaagtagatgaggtcgcataggtaatccatcagcagccagtggtggatgttgtccggggtctggtaggggaaggcccagcgcacgggaatcagccaacagttccaattccaggccatcaccacgaagaacagccataggacatacatcaggttggtcagcgggtcaatgctctggggaaactggtacttcttccaggggcggtgtttgaacttgcagcagagcatgtcgcaatagtgctcctcttccactggctcggcttcagcgggctttgtgtctggagctggctctggggctttcttggctggggagggcttggggctctcctcatcagaggtgacgtcagggtcaatgagtttctccttcactttctctgtccgctccttgaagagcttcaccagctcctggagccggtcgttgatgatggcgctatttgtgctggccgtggaggccgcacggtcctggccatcagtgtccttcggggtggtggggtcagaccaggcaaccactggggactctgctggtgacaacgccttgagctcttcagcctcatcatcctcagagggcagcttcttcctgtgtgtccccgaggctgagcttgggactataagggtgtctgatttggcaggagacggtggcggcaacacggttgagggtggattctcttctgccatgagggggcagctatcagcatcagtatcttccacctgcacttctgggtgctgtttcgtggcaggcactcctgaactggcagcctcggcctcagcctcaggctcctccttggtctccgcccagtcctggggctccttttcagcctcctcttcagccacctcctcggcctcctccttggccttctcttcagcctccttcttggcctcctccccaacttcctcccacagcttctgatctgaagtgctctggggccgggtcccgtcttcttcactctggcccacgcccacctgcgacaccacacagctatccagcagcacctcagtcacctcctcctcttcctcctcctcctcctcttcctcttcctcctcctcatcttctttctcctcttcaatccgggacagctctctgggcatcttctccacagctttgttctcttcttcataagctggaaccacctctgtaccctgtgggctggtactgacatcctggtgggcatcctcccagggcggttcaacctcctctaggacaaggtcaggctccacttgtcctccaggaaggatgctgatggtctgcacatcacatatcccaggggagtcaggctcctgttcccctattttcccatgtagcactggctgcggcaaggccatctccagcctgtgcaggacccatgccaccagcctggcagggtccctggttggtggcagggaggaggtctgggcctgggagccgggctggggctctggagctggtgcctccttgggttcctccttgggctgcagggggatgggtgtgggcagggagggggtctcccgggcctgcagcttgggccccatttcctgggggcgtcctggaggcgctgggtctgaggcagcacctgtagcaactgcaggctcatctctccagacctcagaggatttggggggctgaggaagcactctttccagattctgctccagccacagaagcagccgcagcccaggcctagtgtcttgggcctcaagggcctcattgggttcatctgtgcaccctgtgtccccagtgctgccatgccccaggatctgagccgggtcctccgtgatgctgtgaacaggctgcgggatcaccttctctacgcccttcatgagccaggtcagtaccctgcggctgggactattcatttcagaaatctcagcgccctgggcccggagggatatggtggaagtaagggcagcctccttggtctcctgagggcttgggtctgccacagccacttcctcctccttgaatgactcttcggggggcatggactcggactctgtctcggcctcctcaggattcggttctggttccacctccgcctccatctctggctctggttccacttcctcttcctcctgcatcttggtcttccgaggggtccctgggggctgaggcagcaccctctggacccagcccaacatcctgatgcctgcttagatgccaaccgccagccaggaattgccttcttgctgccactcgtagctggcccctcagacac

SEQ ID NO: 11030 - RNA, 4449 nt, Homo sapiens
  source 1..4449: mol_type = other RNA
ctgaatagctgggactacaggtgcacaccatcacgcctggctattgtttttttgtttgtttttgtttttgtttgagatgaggtctcgctatgttgcccagtctgctctccaactcttggcctccagtgatcctcctgcttcggcttcccaaagcactgggattataggcatgagccaccatgcccggcagtgaagtattttctatccttgaaatgtgttagacaaattcctgaggggaaaccccacacattcaataacactttactttttcagcaaagcttcccatgtattggagcctcattttatccctcacccatgaactttaaaagtggaaaatcattttgttcttaaaaagaggaacagtcaggaaaaggtagggctctcaaatgatagtgagagctcagggactcgaacacttgatgcaacttgtcgagctcaggcccagccccgcgaggagctgagtcggggctggcgtgctggcgggacggtcagagctgcagccactgaggtcacgactacggaaaagcatcttctcttgagccgtgggggaaggtggggcgctggggcgcaggggcgcagcgggcgctggggacacacctgctggaactgcgcgcgggatccgcctcaccccaccttactccgccttctcctccctttcctccggcatcttcaccgacaggatctgctctcccggctccgggcccgggctcatgcagatcctcaccgagtgctcttcgggctcggccggcccctcctcctctccctccggcctcccaagggaggcaggcggtggagagctcggtggagaccccgggggctcggggggcgtccggggcgcgggtgggtcggtggcggcctcctttgggtgcgtgtgctggtctggggcggcggagccttcctctcccttgacgtcttgcgagctcttggcctgttccaccaactcttgctgctttgcagccgcctccagcgcggccagttctttgagccgggcccggaggtgagcaagtttgccgccttttgcccccttgccacccatctttcctgtcatagcgagggcagcgttgaagagctttggggtgcccgcccggggtggaaggatcagcacgctcttctcctccttgggcttattgttgcttctcagcatgcgcctggctttcttccggagtaacttctgagactcaggataatgcaccaaaatctcattcaggtccttcttatccaggatgaagaggttggtaaacccgtgcgccaccacgttggccgtgcgccggttcccgcccccaacagccagcaagcttatttctccaaacacagatccagctttcagcgtcaccagcacagatttcccatcagggccgcccaagacctgcacttgccctgcctggatgatgtacatctcacggccgatctcccccttcttgcacacatagtcgttgggcaggtagacaacagagcgaagcctcttcagcatgtcaaagatcatctgccggtcacagccctgaaagagtgcgactttgctaacgatgttgtagttcacgtcgatggcgaggtccagccgcatcttgtctggaagctgcaccatcagctctgactcatccagcatgccttgcgagtgccaggtgtactcgtaccaggtcttgacgcggttctgcacggacttggggatcttgtagaaattcatgtacttcaccgtgctgtccatgcagctgcggtagtaggtctgtccggcggtggcggcccctaccacatctctcatctgtccgatcatcacagagaaagcaaagacgcccgtgaaataattcagcagctggaagacaatttcaaagagtgtcttggggtcaggcagccccccgatggtgatgagggtcttcacagcaaagtagtaacagcgaatataactgtttcccacgccatcgtaaacccagtgagtggagccgaggccctgataggccgatgcccagtaataaagacaggaattcaaatgcaggctgtagagaaggtaggctgtggtcctgatgaccctgtacacgtaggctttgctgaggatggattccaggcggctgttaaactcgaagaaggccatgtactttaaacagcggggcaggcggaggagggggttcacaccgactttcaaatagagaaaatccaagggcaggaggctgagcaggtccatcttgaagcggcgagacttcaggtagttatttcgcatgtcctttttgtccgtaatgatgtccccgcctctgacaaactgcaggcgtgtctggaacacggtgatgtccaggaagtagatgaggtcgcataggtaatccatcagcagccagtggtggatgttgtccggggtctggtaggggaaggcccagcgcacgggaatcagccaacagttccaattccaggccatcaccacgaagaacagccataggacatacatcaggttggtcagcgggtcaatgctctggggaaactggtacttcttccaggggcggtgtttgaacttgcagcagagcatgtcgcaatagtgctcctcttccactggctcggcttcagcgggctttgtgtctggagctggctctggggctttcttggctggggagggcttggggctctcctcatcagaggtgacgtcagggtcaatgagtttctccttcactttctctgtccgctccttgaagagcttcaccagctcctggagccggtcgttgatgatggcgctatttgtgctggccgtggaggccgcacggtcctggccatcagtgtccttcggggtggtggggtcagaccaggcaaccactggggactctgctggtgacaacgccttgagctcttcagcctcatcatcctcagagggcagcttcttcctgtgtgtccccgaggctgagcttgggactataagggtgtctgatttggcaggagacggtggcggcaacacggttgagggtggattctcttctgccatgagggggcagctatcagcatcagtatcttccacctgcacttctgggtgctgtttcgtggcaggcactcctgaactggcagcctcggcctcagcctcaggctcctccttggtctccgcccagtcctggggctccttttcagcctcctcttcagccacctcctcggcctcctccttggccttctcttcagcctccttcttggcctcctccccaacttcctcccacagcttctgatctgaagtgctctggggccgggtcccgtcttcttcactctggcccacgcccacctgcgacaccacacagctatccagcagcacctcagtcacctcctcctcttcctcctcctcctcctcttcctcttcctcctcctcatcttctttctcctcttcaatccgggacagctctctgggcatcttctccacagctttgttctcttcttcataagctggaaccacctctgtaccctgtgggctggtactgacatcctggtgggcatcctcccagggcggttcaacctcctctaggacaaggtcaggctccacttgtcctccaggaaggatgctgatggtctgcacatcacatatcccaggggagtcaggctcctgttcccctattttcccatgtagcactggctgcggcaaggccatctccagcctgtgcaggacccatgccaccagcctggcagggtccctggttggtggcagggaggaggtctgggcctgggagccgggctggggctctggagctggtgcctccttgggttcctccttgggctgcagggggatgggtgtgggcagggagggggtctcccgggcctgcagcttgggccccatttcctgggggcgtcctggaggcgctgtagcaactgcaggctcatctctccagacctcagaggatttggggggctgaggaagcactctttccagattctgctccagccacagaagcagccgcagcccaggcctagtgtcttgggcctcaagggcctcattgggttcatctgtgcaccctgtgtccccagtgctgccatgccccaggatctgagccgggtcctccgtgatgctgtgaacaggctgcgggatcaccttctctacgcccttcatgagccaggtcagtaccctgcggctgggactattcatttcagaaatctcagcgccctgggcccggagggatatggtggaagtaagggcagcctccttggtctcctgagggcttgggtctgccacagccacttcctcctccttgaatgactcttcggggggcatggactcggactctgtctcggcctcctcaggattcggttctggttccacctccgcctccatctctggctctggttccacttcctcttcctcctgcatcttggtcttccgaggggtccctgggggctgaggcagcaccctctggacccagcccaacatcctgatgcctgcttagatgccaaccgccagccaggaattgccttcttgctgccactcgtagctggcccctcagacac

SEQ ID NO: 11031 - RNA, 2731 nt, Homo sapiens
  source 1..2731: mol_type = other RNA
ctgaatagctgggactacaggtgcacactactccacccagctaattttcaaatattttgtagagacagcgtcttgctatgttgcttagggtggtctcaaactcctgggctcaagcagtcctcctgccttggcctcccaaagtgctgcgattacaggcatgaaccaccgtgcccagccttttctgttttttggtttttcgtttttgagacagagtctcactctgttgcccaggctggagtgtggtggcacaatctcagctcaccgcaacctctgcctcacgggctcaagtgattctcatgcttcatcctcccaagtagctgggattacaggcacatgccatcatgcctagctaacttttgtatttttggtagagacgaggtttcaccatgttggccaggctgtctcaaactcctgacctcagatgatccgcccacctcagcctcccaaagtgctgggactacaggcatgaaccaccgcacccggcccaaggagtttgccttttcattttgcactgggccctggatattacatagctgaccttgtcttcaggactaggaaaaggaccgatagaatcctgtgttccttttgaattaatctacatttctttgacaacaagctggacataggcttcatgaagtacagggggctccaggaatactttgttctgaaatccaagaatcctcactgtatcctttacccaagctctggcatatgtcatcatgactttggttcccttggggcaaagagcatacttttggcctgaatggacattgagtgtgggggtgcttaacacctctgaacaggtcttgtccacttttgagttggagggcaggtcagctaggtgtgcacttccaaaagagccctcactgtccaaggtgcagttgtaatccaggaaggaaatgaggtccatgatgtgccactatgtggagaactcacaggttatcacaacactgaaactcttgatgaatgattactggaggagggagtttacatcgtgtcaggccctacactatggagtgtagggatgccacccttggttcccattgtccaaaaacaaaacccaggaacttccacatcttactgtccttcacattggtgtggaaggctttgaagaatctgctgtcctgatgagcgccttgtctcaccacaaaaggctacaacagggatatggcatcaattggatcctcatccagcttgaaataaaccgtggaagctgcttttcctcaggacccgatagagggtgaagttctgggcttggtagagactgaagcagactggcacatcagtggtcacgattggctttatgaggatcttctacttctaaatcccaaacataaagtttgccaacttgattgcccaatgcaagcatcttttgccagaaatccatagaaaacctcatgtaccaaatgtcacactggctgtaatcaaatcgcccaagaatagtcacattagattcactgggtttaattttatctatatcatcttccatcttgccaggtttccagcacacaatggcattttcacaagaagcacttagaacttcatctctgtgcccttctacgcctccaaatattgccaccagagtgtccgtctggatattccataatcgtaaagcatgatctttacttactgacaggagaagatttggatctcttggatggaatttcagctcattgatagcatttccatggccaacatagtgctttatacactgcattgttataggatttattatcctaattatgcctctagatccagctacagccagcagaggatggctcgtattgctatcataggtccatgcacaagtgtaaaagttttcatcagcatcagcatccacgtaagattgcaacaaccggatttctccttgtgaatgacattcatacaaggtaactctgttgcttcctacagttgcaaacactaatggatctccttctttactgtgccagttaaactgaactccaaacaatggttggttatgatcttccttgagactatttacacatttgaaagaatatttgcatttctttgacttccattttccctttccccaacttttccttccaggtgcatttggcgtgtttgtaggtgtatcagggcgttcagtgtttgtaccactttctatactgacagcgtcatcattctcgtctccagagaggtctggattgctgttctcgtcactgctcagcttctgcttcttggccgcaggcatgtctgttcccgccggcgcagtcgacacttccctctcggacatattcctccgcctccctccaggttcctgccgcctggggcggggcctccgccacaccgccgtcaagcaagcccggcccgagcttgccgcaaagttgccgctgccgccgccacctccaccgccccccccactgtcgcaaatcgcgcccagccgccgaggcgggcgtgcgtgcgaccccgccacactgctgaaaaaggggcgcgcgcgcgcgccctcccgcgcggcttcctggctccttcccttccccaactcccgtcttgcccttttcccgccgccctcccggcagtctacacgatgtaaggtccgttggattaagagggcagtattaagtatgtctcccttcccaccaccgcctcgagaagaggcgaaactcaaagggatgctccctcacccccttcctccttccaaagacgtttcagccgcaattggcccgttccttcgatctccgacccgctgctagggagcgaaagtctgtggaat

SEQ ID NO: 11032 - RNA, 3046 nt, Homo sapiens
  source 1..3046: mol_type = other RNA
ctgaatagctgggactacaggtgcacactactccacccagctaattttcaaatattttgtagagacagcgtcttgctatgttgcttagggtggtctcaaactcctgggctcaagcagtcctcctgccttggcctcccaaagtgctgcgattacaggcatgaaccaccgtgcccagccttttctgttttttggtttttcgtttttgagacagagtctcactctgttgcccaggctggagtgtggtggcacaatctcagctcaccgcaacctctgcctcacgggctcaagtgattctcatgcttcatcctcccaagtagctgggattacaggcacatgccatcatgcctagctaacttttgtatttttggtagagacgaggtttcaccatgttggccaggctgtctcaaactcctgacctcagatgatccgcccacctcagcctcccaaagtgctgggactacaggcatgaaccaccgcacccggcccaaggagtttgccttttcattttgcactgggccctggatattacatagctgaccttgtcttcaggactaggaaaaggaccgatagaatcctgtgttccttttgaattaatctacatttctttgacaacaagctggacataggcttcatgaagtacagggggctccaggaatactttgttctgaaatccaagaatcctcactgtatcctttacccaagctctggcatatgtcatcatgactttggttcccttggggcaaagagcatacttttggcctgaatggacattgagtgtgggggtgcttaacacctctgaacaggtcttgtccacttttgagttggagggcaggtcagctaggtgtgcacttccaaaagagccctcactgtccaaggtgcagttgtaatccaggaaggaaatgaggtccatgatgtgccactatgtggagaactcacaggttatcacaacactgaaactcttgatgaatgattactggaggagggagtttacatcgtgtcaggccctacactatggagtgtagggatgccacccttggttcccattgtccaaaaacaaaacccaggaacttccacatcttactgtccttcacattggtgtggaaggctttgaagaatctgctgtcctgatgagcgccttgtctcaccacaaaaggctacaacagggatatggcatcaattggatcctcatccagcttgaaataaaccgtggaagctgcttttcctcaggacccgatagagggtgaagttctgggcttggtagagactgaagcagactggcacatcagtggtcacgattggctttatgaggatcttctacttctaaatcccaaacataaagtttgccaacttgattgcccaatgcaagcatcttttgccagaaatccatagaaaacctcatgtaccaaatgtcacactggctgtaatcaaatcgcccaagaatagtcacattagattcactgggtttaattttatctatatcatcttccatcttgccaggtttccagcacacaatggcattttcacaagacaaatgctggcgaagattcggagacactggatctctcatacattgctggtgggaatgtaaaatggcacggccactcttagaaagtatcaaatcgcctaaccatcgcacacaatcaacataattcctatgtatgtctctggtagaaaaatcaggaaaatggattttctgagaaataaatggcctgttagttttatttggattataatcataagattccttaattgcattcatcattctctttgaattgatcctccaaagtttaagagaatgatccataccacaggacattattttttcacccaaaagatcataatcagcacttagaacttcatctctgtgcccttctacgcctccaaatattgccaccagagtgtccgtctggatattccataatcgtaaagcatgatctttacttactgacaggagaagatttggatctcttggatggaatttcagctcattgatagcatttccatggccaacatagtgctttatacactgcattgttataggatttattatcctaattatgcctctagatccagctacagccagcagaggatggctcgtattgctatcataggtccatgcacaagtgtaaaagttttcatcagcatcagcatccacgtaagattgcaacaaccggatttctccttgtgaatgacattcatacaaggtaactctgttgcttcctacagttgcaaacactaatggatctccttctttactgtgccagttaaactgaactccaaacaatggttggttatgatcttccttgagactatttacacatttgaaagaatatttgcatttctttgacttccattttccctttccccaacttttccttccaggtgcatttggcgtgtttgtaggtgtatcagggcgttcagtgtttgtaccactttctatactgacagcgtcatcattctcgtctccagagaggtctggattgctgttctcgtcactgctcagcttctgcttcttggccgcaggcatgtctgttcccgccggcgcagtcgacacttccctctcggacatattcctccgcctccctccaggttcctgccgcctggggcggggcctccgccacaccgccgtcaagcaagcccggcccgagcttgccgcaaagttgccgctgccgccgccacctccaccgccccccccactgtcgcaaatcgcgcccagccgccgaggcgggcgtgcgtgcgaccccgccacactgctgaaaaaggggcgcgcgcgcgcgccctcccgcgcggcttcctggctccttcccttccccaactcccgtcttgcccttttcccgccgccctcccggcagtctacacgatgtaaggtccgttggattaagagggcagtattaagtatgtctcccttcccaccaccgcctcgagaagaggcgaaactcaaagggatgctccctcacccccttcctccttccaaagacgtttcagccgcaattggcccgttccttcgatctccgacccgctgctagggagcgaaagtctgtggaat

SEQ ID NO: 11033 - RNA, 2337 nt, Homo sapiens
  source 1..2337: mol_type = other RNA
ctgaatagctgggactacaggtgcacagcaccatacctggctaatgtttgtattttttgtagagatggtgtttcaccacgttacctaggttgaccttgaactcctgggctcaagtgatccgcttgccttggcttcccaaagtgctgggattacaggtgtgagccaccgcgccaggccttgggtaattctttgttgcagtagactgttctgtgtcctgtggtgggtttaacagcagcactcactctgcctgctagatgccagtagcaacctccttcataagctgtgatagccagaaatatccccagacattgtcaaatgtctcctgggggtaaaattgcctctggttgagaaccactggtatattgtctatgtctccagttagaagggcagttccatgagagtgaagaccccacgtccaagttcctcagggccctgatgacctcagcctggcattcactcttccatgcagctgatcctccccaagccctggactgggccgcaggctacctgagaagcacatcaaagcgtttgttctacaggaccctcgtctgtgggcttgtgcagcttggggccagggatggtggcctactggcctttgcactgccagtacccacccaggctttgctttcagggtggtcagaaaatgattactgggggaacacatgacagaaaagcaggaagggggcctcttggtgctgtgagctgaccagtgcacagtgttggtccttctcgacagggatgacttctactttttggaagggagagttcagactttattagataccttaaggctggccctggggaaaaccgtggctggcttcaccatcctcctaataggaagaggcagtgaggagaacagtagtctggggaaggtgggagccccaactgaggggcctgcacccagcccctcagatccgcctcccctcccatgtcactccagctcttttgggatgatcacatggtgagaatctgctttgaagatatgaagggcttcatggaggcttccaaggcagactggtagtcctgcagcgggacctgggagcaggcaggggctgtgagctggcctcggcggatgagatcgcacagtgtgaggatcagctccttgaactggtctggactgtgatccttcttccactgggacaaccaaaagcctcgaagtttgagatccttaaaaatgagcaggctcacagaggctacgacgggctgcttggccatccccccataggttaccatggttcctccacgcctggacttggctcgaactggcgatgggactcagtcacttgatggtcctcccagctaaagacctggagagctctggcgagctggacctgcaggcccaagggacttacgctaactgccgcagcagctctgtggagcttttcccaccaacacagttgagagcaagccgtggctggggcatgtccttaaagaagtttttcatttcgggccttcttagctcctcttctgtgatgacatgctcagcccccagactcttcagtctgtcactcagcttctggatatcaggtctgtctcggaccacattgatggttcttaggcccagggctgcggcgatctggatgactgcttgccccactccgctgttggatgcattctggatgacagaatcccctggctgcagttgctcgaagtccatcaacatcctgtaggctgtgcagggattgacacccagggtggcagcgctctgaagagggatgtcactcggaacttggatcagtgcttcctcgctgaacacagcctcggtccgccaggttcctaaaccagcatttgctggaatcacccagtctcctggcttcagcccggtcacattgctgcccaccgctaccacctgtgcaacaccttcgttccctccaacagcaggcagttcaggaaggaatccgtagtttccttggatcatatttatgtcagatggattgataggggccgccagcatcttcacacggacatctgatcctctcacagcagctagctccaggttcttgagtctaagcacaaagccaaacggagatgttcatgtcatccaggctagaatgggtgtttcgctcaaatcatctcctcaaagtaggtcaggcaacatttctgagctgccatgtgtgcccaggaattacggtttcgacgaccttggctggatccccgtggtgcccatagacaagcgcccggacccgggcaggctcggcggatgcggagtaggaggaggcggcaggtccgtgacagccagaagctgggagcagcccccgccactgccgggcgggggttcgcacccgccacagggtactgcagacccacatgctcgctccaaccaacacagagcctgac

SEQ ID NO: 11034 - RNA, 2209 nt, Homo sapiens
  source 1..2209: mol_type = other RNA
ctgaatagctgggactacaggtgcacagcaccatacctggctaatgtttgtattttttgtagagatggtgtttcaccacgttacctaggttgaccttgaactcctgggctcaagtgatccgcttgccttggcttcccaaagtgctgggattacaggtgtgagccaccgcgccaggccttgggtaattctttgttgcagtagactgttctgtgtcctgtggtgggtttaacagcagcactcactctgcctgctagatgccagtagcaacctccttcataagctgtgatagccagaaatatccccagacattgtcaaatgtctcctgggggtaaaattgcctctggttgagaaccactggtatattgtctatgtctccagttagaagggcagttccatgagagtgaagaccccacgtccaagttcctcagggccctgatgacctcagcctggcattcactcttccatgcagctgatcctccccaagccctggactgggccgcaggctacctgagaagcacatcaaagcgtttgttctacaggaccctcgtctgtgggcttgtgcagcttggggccagggatggtggcctactggcctttgcactgccagtacccacccaggctttgctttcagggtggtcagaaaatgattactgggggaacacatgacagaaaagcaggaagggggcctcttggtgctgtgagctgaccagtgcacagtgttggtccttctcgacagggatgacttctactttttggaagggagagttcagactttattagataccttaaggctggccctggggaaaaccgtggctggcttcaccatcctcctaataggaagaggcagtgaggagaacagtagtctggggaaggtgggagccccaactgaggggcctgcacccagcccctcagatccgcctcccctcccatgtcactccagctcttttgggatgatcacatggtgagaatctgctttgaagatatgaagggcttcatggaggcttccaaggcagactggtagtcctgcagcgggacctgggagcaggcaggggctgtgagctggcctcggcggatgagatcgcacagtgtgaggatcagctccttgaactggtctggactgtgatccttcttccactgggacaaccaaaagcctcgaagtttgagatccttaaaaatgagcaggctcacagaggctacgacgggctgcttggccatccccccataggttaccatggttcctccacgcgctaactgccgcagcagctctgtggagcttttcccaccaacacagttgagagcaagccgtggctggggcatgtccttaaagaagtttttcatttcgggccttcttagctcctcttctgtgatgacatgctcagcccccagactcttcagtctgtcactcagcttctggatatcaggtctgtctcggaccacattgatggttcttaggcccagggctgcggcgatctggatgactgcttgccccactccgctgttggatgcattctggatgacagaatcccctggctgcagttgctcgaagtccatcaacatcctgtaggctgtgcagggattgacacccagggtggcagcgctctgaagagggatgtcactcggaacttggatcagtgcttcctcgctgaacacagcctcggtccgccaggttcctaaaccagcatttgctggaatcacccagtctcctggcttcagcccggtcacattgctgcccaccgctaccacctgtgcaacaccttcgttccctccaacagcaggcagttcaggaaggaatccgtagtttccttggatcatatttatgtcagatggattgataggggccgccagcatcttcacacggacatctgatcctctcacagcagctagctccaggttcttgagtacagtagatgctgaagaaatgacagctgttatcagttgtaggaatatccaaggaaacctctggaacaattccctggttatacctctgaaaagaatcactgagtcatcgacgaccttggctggatccccgtggtgcccatagacaagcgcccggacccgggcaggctcggcggatgcggagtaggaggaggcggcaggtccgtgacagccagaagctgggagcagcccccgccactgccgggcgggggttcgcacccgccacagggtactgcagacccacatgctcgctccaaccaacacagagcctgac

SEQ ID NO: 11035 - RNA, 2435 nt, Homo sapiens
  source 1..2435: mol_type = other RNA
ctgaatagctgggactacaggtgcacagcaccatacctggctaatgtttgtattttttgtagagatggtgtttcaccacgttacctaggttgaccttgaactcctgggctcaagtgatccgcttgccttggcttcccaaagtgctgggattacaggtgtgagccaccgcgccaggccttgggtaattctttgttgcagtagactgttctgtgtcctgtggtgggtttaacagcagcactcactctgcctgctagatgccagtagcaacctccttcataagctgtgatagccagaaatatccccagacattgtcaaatgtctcctgggggtaaaattgcctctggttgagaaccactggtatattgtctatgtctccagttagaagggcagttccatgagagtgaagaccccacgtccaagttcctcagggccctgatgacctcagcctggcattcactcttccatgcagctgatcctccccaagccctggactgggccgcaggctacctgagaagcacatcaaagcgtttgttctacaggaccctcgtctgtgggcttgtgcagcttggggccagggatggtggcctactggcctttgcactgccagtacccacccaggctttgctttcagggtggtcagaaaatgattactgggggaacacatgacagaaaagcaggaagggggcctcttggtgctgtgagctgaccagtgcacagtgttggtccttctcgacagggatgacttctactttttggaagggagagttcagactttattagataccttaaggctggccctggggaaaaccgtggctggcttcaccatcctcctaataggaagaggcagtgaggagaacagtagtctggggaaggtgggagccccaactgaggggcctgcacccagcccctcagatccgcctcccctcccatgtcactccagctcttttgggatgatcacatggtgagaatctgctttgaagatatgaagggcttcatggaggcttccaaggcagactggtagtcctgcagcgggacctgggagcaggcaggggctgtgagctggcctcggcggatgagatcgcacagtgtgaggatcagctccttgaactggtctggactgtgatccttcttccactgggacaaccaaaagcctcgaagtttgagatccttaaaaatgagcaggctcacagaggctacgacgggctgcttggccatccccccataggttaccatggttcctccacgcgctaactgccgcagcagctctgtggagcttttcccaccaacacagttgagagcaagccgtggctggggcatgtccttaaagaagtttttcatttcgggccttcttagctcctcttctgtgatgacatgctcagcccccagactcttcagtctgtcactcagcttctggatatcaggtctgtctcggaccacattgatggttcttaggcccagggctgcggcgatctggatgactgcttgccccactccgctgttggatgcattctggatgacagaatcccctggctgcagttgctcgaagtccatcaacatcctgtaggctgtgcagggattgacacccagggtggcagcgctctgaagagggatgtcactcggaacttggatcagtgcttcctcgctgaacacagcctcggtccgccaggttcctaaaccagcatttgctggaatcacccagtctcctggcttcagcccggtcacattgctgcccaccgctaccacctgtgcaacaccttcgttccctccaacagcaggcagttcaggaaggaatccgtagtttccttggatcatatttatgtcagatggattgataggggccgccagcatcttcacacggacatctgatcctctcacagcagctagctccaggttcttgagtacagtagatgctgaagaaatgacagctgttatcagttgtaggaatatccaaggaaacctctggaacaattccctggttatacctctgtagtcccagctacttgggaggctgaggaaggagagttgcttgtgctcaggagttcaaggctattgtgtaccatcatcacacctgtgaatgaccactgcactctagcctgggcaacaggagacccgttcacgtcctccgtgaatgtaatggcgccatgcaactcgaggggatgccactgtcctcaatcaacagatcccagcctggataaggtcacaatggctcctttgaggccaaggctgtacactcgacgaccttggctggatccccgtggtgcccatagacaagcgcccggacccgggcaggctcggcggatgcggagtaggaggaggcggcaggtccgtgacagccagaagctgggagcagcccccgccactgccgggcgggggttcgcacccgccacagggtactgcagacccacatgctcgctccaaccaacacagagcctgac

SEQ ID NO: 11036 - RNA, 2188 nt, Homo sapiens
  source 1..2188: mol_type = other RNA
ctgaatagctgggactacaggtgcacagcaccatacctggctaatgtttgtattttttgtagagatggtgtttcaccacgttacctaggttgaccttgaactcctgggctcaagtgatccgcttgccttggcttcccaaagtgctgggattacaggtgtgagccaccgcgccaggccttgggtaattctttgttgcagtagactgttctgtgtcctgtggtgggtttaacagcagcactcactctgcctgctagatgccagtagcaacctccttcataagctgtgatagccagaaatatccccagacattgtcaaatgtctcctgggggtaaaattgcctctggttgagaaccactggtatattgtctatgtctccagttagaagggcagttccatgagagtgaagaccccacgtccaagttcctcagggccctgatgacctcagcctggcattcactcttccatgcagctgatcctccccaagccctggactgggccgcaggctacctgagaagcacatcaaagcgtttgttctacaggaccctcgtctgtgggcttgtgcagcttggggccagggatggtggcctactggcctttgcactgccagtacccacccaggctttgctttcagggtggtcagaaaatgattactgggggaacacatgacagaaaagcaggaagggggcctcttggtgctgtgagctgaccagtgcacagtgttggtccttctcgacagggatgacttctactttttggaagggagagttcagactttattagataccttaaggctggccctggggaaaaccgtggctggcttcaccatcctcctaataggaagaggcagtgaggagaacagtagtctggggaaggtgggagccccaactgaggggcctgcacccagcccctcagatccgcctcccctcccatgtcactccagctcttttgggatgatcacatggtgagaatctgctttgaagatatgaagggcttcatggaggcttccaaggcagactggtagtcctgcagcgggacctgggagcaggcaggggctgtgagctggcctcggcggatgagatcgcacagtgtgaggatcagctccttgaactggtctggactgtgatccttcttccactgggacaaccaaaagcctcgaagtttgagatccttaaaaatgagcaggctcacagaggctacgacgggctgcttggccatccccccataggttaccatggttcctccacgcgctaactgccgcagcagctctgtggagcttttcccaccaacacagttgagagcaagccgtggctggggcatgtccttaaagaagtttttcatttcgggccttcttagctcctcttctgtgatgacatgctcagcccccagactcttcagtctgtcactcagcttctggatatcaggtctgtctcggaccacattgatggttcttaggcccagggctgcggcgatctggatgactgcttgccccactccgctgttggatgcattctggatgacagaatcccctggctgcagttgctcgaagtccatcaacatcctgtaggctgtgcagggattgacacccagggtggcagcgctctgaagagggatgtcactcggaacttggatcagtgcttcctcgctgaacacagcctcggtccgccaggttcctaaaccagcatttgctggaatcacccagtctcctggcttcagcccggtcacattgctgcccaccgctaccacctgtgcaacaccttcgttccctccaacagcaggcagttcaggaaggaatccgtagtttccttggatcatatttatgtcagatggattgataggggccgccagcatcttcacacggacatctgatcctctcacagcagctagctccaggttcttgagtacagtagatgctgaagaaatgacagctgttatcagttgtaggaatatccaaggaaacctctggaacaattccctggttataccttcgacgaccttggctggatccccgtggtgcccatagacaagcgcccggacccgggcaggctcggcggatgcggagtaggaggaggcggcaggtccgtgacagccagaagctgggagcagcccccgccactgccgggcgggggttcgcacccgccacagggtactgcagacccacatgctcgctccaaccaacacagagcctgac

SEQ ID NO: 11037 - RNA, 2225 nt, Homo sapiens
  source 1..2225: mol_type = other RNA
ctgaatagctgggactacaggtgcacagcaccatacctggctaatgtttgtattttttgtagagatggtgtttcaccacgttacctaggttgaccttgaactcctgggctcaagtgatccgcttgccttggcttcccaaagtgctgggattacaggtgtgagccaccgcgccaggccttgggtaattctttgttgcagtagactgttctgtgtcctgtggtgggtttaacagcagcactcactctgcctgctagatgccagtagcaacctccttcataagctgtgatagccagaaatatccccagacattgtcaaatgtctcctgggggtaaaattgcctctggttgagaaccactggtatattgtctatgtctccagttagaagggcagttccatgagagtgaagaccccacgtccaagttcctcagggccctgatgacctcagcctggcattcactcttccatgcagctgatcctccccaagccctggactgggccgcaggctacctgagaagcacatcaaagcgtttgttctacaggaccctcgtctgtgggcttgtgcagcttggggccagggatggtggcctactggcctttgcactgccagtacccacccaggctttgctttcagggtggtcagaaaatgattactgggggaacacatgacagaaaagcaggaagggggcctcttggtgctgtgagctgaccagtgcacagtgttggtccttctcgacagggatgacttctactttttggaagggagagttcagactttattagataccttaaggctggccctggggaaaaccgtggctggcttcaccatcctcctaataggaagaggcagtgaggagaacagtagtctggggaaggtgggagccccaactgaggggcctgcacccagcccctcagatccgcctcccctcccatgtcactccagctcttttgggatgatcacatggtgagaatctgctttgaagatatgaagggcttcatggaggcttccaaggcagactggtagtcctgcagcgggacctgggagcaggcaggggctgtgagctggcctcggcggatgagatcgcacagtgtgaggatcagctccttgaactggtctggactgtgatccttcttccactgggacaaccaaaagcctcgaagtttgagatccttaaaaatgagcaggctcacagaggctacgacgggctgcttggccatccccccataggttaccatggttcctccacgcgctaactgccgcagcagctctgtggagcttttcccaccaacacagttgagagcaagccgtggctggggcatgtccttaaagaagtttttcatttcgggccttcttagctcctcttctgtgatgacatgctcagcccccagactcttcagtctgtcactcagcttctggatatcaggtctgtctcggaccacattgatggttcttaggcccagggctgcggcgatctggatgactgcttgccccactccgctgttggatgcattctggatgacagaatcccctggctgcagttgctcgaagtccatcaacatcctgtaggctgtgcagggattgacacccagggtggcagcgctctgaagagggatgtcactcggaacttggatcagtgcttcctcgctgaacacagcctcggtccgccaggttcctaaaccagcatttgctggaatcacccagtctcctggcttcagcccggtcacattgctgcccaccgctaccacctgtgcaacaccttcgttccctccaacagcaggcagttcaggaaggaatccgtagtttccttggatcatatttatgtcagatggattgataggggccgccagcatcttcacacggacatctgatcctctcacagcagctagctccaggttcttgagtcgttcacgtcctccgtgaatgtaatggcgccatgcaactcgaggggatgccactgtcctcaatcaacagatcccagcctggataaggtcacaatggctcctttgaggccaaggctgtacactcgacgaccttggctggatccccgtggtgcccatagacaagcgcccggacccgggcaggctcggcggatgcggagtaggaggaggcggcaggtccgtgacagccagaagctgggagcagcccccgccactgccgggcgggggttcgcacccgccacagggtactgcagacccacatgctcgctccaaccaacacagagcctgac

SEQ ID NO: 11038 - RNA, 2436 nt, Homo sapiens
  source 1..2436: mol_type = other RNA
ctgaatagctgggactacaggtgcacagcaccatacctggctaatgtttgtattttttgtagagatggtgtttcaccacgttacctaggttgaccttgaactcctgggctcaagtgatccgcttgccttggcttcccaaagtgctgggattacaggtgtgagccaccgcgccaggccttgggtaattctttgttgcagtagactgttctgtgtcctgtggtgggtttaacagcagcactcactctgcctgctagatgccagtagcaacctccttcataagctgtgatagccagaaatatccccagacattgtcaaatgtctcctgggggtaaaattgcctctggttgagaaccactggtatattgtctatgtctccagttagaagggcagttccatgagagtgaagaccccacgtccaagttcctcagggccctgatgacctcagcctggcattcactcttccatgcagctgatcctccccaagccctggactgggccgcaggctacctgagaagcacatcaaagcgtttgttctacaggaccctcgtctgtgggcttgtgcagcttggggccagggatggtggcctactggcctttgcactgccagtacccacccaggctttgctttcagggtggtcagaaaatgattactgggggaacacatgacagaaaagcaggaagggggcctcttggtgctgtgagctgaccagtgcacagtgttggtccttctcgacagggatgacttctactttttggaagggagagttcagactttattagataccttaaggctggccctggggaaaaccgtggctggcttcaccatcctcctaataggaagaggcagtgaggagaacagtagtctggggaaggtgggagccccaactgaggggcctgcacccagcccctcagatccgcctcccctcccatgtcactccagctcttttgggatgatcacatggtgagaatctgctttgaagatatgaagggcttcatggaggcttccaaggcagactggtagtcctgcagcgggacctgggagcaggcaggggctgtgagctggcctcggcggatgagatcgcacagtgtgaggatcagctccttgaactggtctggactgtgatccttcttccactgggacaaccaaaagcctcgaagtttgagatccttaaaaatgagcaggctcacagaggctacgacgggctgcttggccatccccccataggttaccatggttcctccacgcgctaactgccgcagcagctctgtggagcttttcccaccaacacagttgagagcaagccgtggctggggcatgtccttaaagaagtttttcatttcgggccttcttagctcctcttctgtgatgacatgctcagcccccagactcttcagtctgtcactcagcttctggatatcaggtctgtctcggaccacattgatggttcttaggcccagggctgcggcgatctggatgactgcttgccccactccgctgttggatgcattctggatgacagaatcccctggctgcagttgctcgaagtccatcaacatcctgtaggctgtgcagggattgacacccagggtggcagcgctctgaagagggatgtcactcggaacttggatcagtgcttcctcgctgaacacagcctcggtccgccaggttcctaaaccagcatttgctggaatcacccagtctcctggcttcagcccggtcacattgctgcccaccgctaccacctgtgcaacaccttcgttccctccaacagcaggcagttcaggaaggaatccgtagtttccttggatcatatttatgtcagatggattgataggggccgccagcatcttcacacggacatctgatcctctcacagcagctagctccaggttcttgagtctaagcacaaagccaaacggagatgttcatgtcatccaggctagaatgggtgtttcgctcaaatcatctcctcaaagtaggtcaggcaacatttctgagctgccatgtgtgcccaggaattacggttacagtagatgctgaagaaatgacagctgttatcagttgtaggaatatccaaggaaacctctggaacaattccctggttatacctcgttcacgtcctccgtgaatgtaatggcgccatgcaactcgaggggatgccactgtcctcaatcaacagatcccagcctggataaggtcacaatggctcctttgaggccaaggctgtacactcgacgaccttggctggatccccgtggtgcccatagacaagcgcccggacccgggcaggctcggcggatgcggagtaggaggaggcggcaggtccgtgacagccagaagctgggagcagcccccgccactgccgggcgggggttcgcacccgccacagggtactgcagacccacatgctcgctccaaccaacacagagcctgac

SEQ ID NO: 11039 - RNA, 2231 nt, Homo sapiens
  source 1..2231: mol_type = other RNA
ctgaatagctgggactacaggtgcacagcaccatacctggctaatgtttgtattttttgtagagatggtgtttcaccacgttacctaggttgaccttgaactcctgggctcaagtgatccgcttgccttggcttcccaaagtgctgggattacaggtgtgagccaccgcgccaggccttgggtaattctttgttgcagtagactgttctgtgtcctgtggtgggtttaacagcagcactcactctgcctgctagatgccagtagcaacctccttcataagctgtgatagccagaaatatccccagacattgtcaaatgtctcctgggggtaaaattgcctctggttgagaaccactggtatattgtctatgtctccagttagaagggcagttccatgagagtgaagaccccacgtccaagttcctcagggccctgatgacctcagcctggcattcactcttccatgcagctgatcctccccaagccctggactgggccgcaggctacctgagaagcacatcaaagcgtttgttctacaggaccctcgtctgtgggcttgtgcagcttggggccagggatggtggcctactggcctttgcactgccagtacccacccaggctttgctttcagggtggtcagaaaatgattactgggggaacacatgacagaaaagcaggaagggggcctcttggtgctgtgagctgaccagtgcacagtgttggtccttctcgacagggatgacttctactttttggaagggagagttcagactttattagataccttaaggctggccctggggaaaaccgtggctggcttcaccatcctcctaataggaagaggcagtgaggagaacagtagtctggggaaggtgggagccccaactgaggggcctgcacccagcccctcagatccgcctcccctcccatgtcactccagctcttttgggatgatcacatggtgagaatctgctttgaagatatgaagggcttcatggaggcttccaaggcagactggtagtcctgcagcgggacctgggagcaggcaggggctgtgagctggcctcggcggatgagatcgcacagtgtgaggatcagctccttgaactggtctggactgtgatccttcttccactgggacaaccaaaagcctcgaagtttgagatccttaaaaatgagcaggctcacagaggctacgacgggctgcttggccatccccccataggttaccatggttcctccacgcgctaactgccgcagcagctctgtggagcttttcccaccaacacagttgagagcaagccgtggctggggcatgtccttaaagaagtttttcatttcgggccttcttagctcctcttctgtgatgacatgctcagcccccagactcttcagtctgtcactcagcttctggatatcaggtctgtctcggaccacattgatggttcttaggcccagggctgcggcgatctggatgactgcttgccccactccgctgttggatgcattctggatgacagaatcccctggctgcagttgctcgaagtccatcaacatcctgtaggctgtgcagggattgacacccagggtggcagcgctctgaagagggatgtcactcggaacttggatcagtgcttcctcgctgaacacagcctcggtccgccaggttcctaaaccagcatttgctggaatcacccagtctcctggcttcagcccggtcacattgctgcccaccgctaccacctgtgcaacaccttcgttccctccaacagcaggcagttcaggaaggaatccgtagtttccttggatcatatttatgtcagatggattgataggggccgccagcatcttcacacggacatctgatcctctcacagcagctagctccaggttcttgagtctaagcacaaagccaaacggagatgttcatgtcatccaggctagaatgggtgtttcgctcaaatcatctcctcaaagtaggtcaggcaacatttctgagctgccatgtgtgcccaggaattacggtttcgacgaccttggctggatccccgtggtgcccatagacaagcgcccggacccgggcaggctcggcggatgcggagtaggaggaggcggcaggtccgtgacagccagaagctgggagcagcccccgccactgccgggcgggggttcgcacccgccacagggtactgcagacccacatgctcgctccaaccaacacagagcctgac

SEQ ID NO: 11040 - RNA, 2313 nt, Homo sapiens
  source 1..2313: mol_type = other RNA
ctgaatagctgggactacaggtgcacagcaccatacctggctaatgtttgtattttttgtagagatggtgtttcaccacgttacctaggttgaccttgaactcctgggctcaagtgatccgcttgccttggcttcccaaagtgctgggattacaggtgtgagccaccgcgccaggccttgggtaattctttgttgcagtagactgttctgtgtcctgtggtgggtttaacagcagcactcactctgcctgctagatgccagtagcaacctccttcataagctgtgatagccagaaatatccccagacattgtcaaatgtctcctgggggtaaaattgcctctggttgagaaccactggtatattgtctatgtctccagttagaagggcagttccatgagagtgaagaccccacgtccaagttcctcagggccctgatgacctcagcctggcattcactcttccatgcagctgatcctccccaagccctggactgggccgcaggctacctgagaagcacatcaaagcgtttgttctacaggaccctcgtctgtgggcttgtgcagcttggggccagggatggtggcctactggcctttgcactgccagtacccacccaggctttgctttcagggtggtcagaaaatgattactgggggaacacatgacagaaaagcaggaagggggcctcttggtgctgtgagctgaccagtgcacagtgttggtccttctcgacagggatgacttctactttttggaagggagagttcagactttattagataccttaaggctggccctggggaaaaccgtggctggcttcaccatcctcctaataggaagaggcagtgaggagaacagtagtctggggaaggtgggagccccaactgaggggcctgcacccagcccctcagatccgcctcccctcccatgtcactccagctcttttgggatgatcacatggtgagaatctgctttgaagatatgaagggcttcatggaggcttccaaggcagactggtagtcctgcagcgggacctgggagcaggcaggggctgtgagctggcctcggcggatgagatcgcacagtgtgaggatcagctccttgaactggtctggactgtgatccttcttccactgggacaaccaaaagcctcgaagtttgagatccttaaaaatgagcaggctcacagaggctacgacgggctgcttggccatccccccataggttaccatggttcctccacgcgctaactgccgcagcagctctgtggagcttttcccaccaacacagttgagagcaagccgtggctggggcatgtccttaaagaagtttttcatttcgggccttcttagctcctcttctgtgatgacatgctcagcccccagactcttcagtctgtcactcagcttctggatatcaggtctgtctcggaccacattgatggttcttaggcccagggctgcggcgatctggatgactgcttgccccactccgctgttggatgcattctggatgacagaatcccctggctgcagttgctcgaagtccatcaacatcctgtaggctgtgcagggattgacacccagggtggcagcgctctgaagagggatgtcactcggaacttggatcagtgcttcctcgctgaacacagcctcggtccgccaggttcctaaaccagcatttgctggaatcacccagtctcctggcttcagcccggtcacattgctgcccaccgctaccacctgtgcaacaccttcgttccctccaacagcaggcagttcaggaaggaatccgtagtttccttggatcatatttatgtcagatggattgataggggccgccagcatcttcacacggacatctgatcctctcacagcagctagctccaggttcttgagtctacacagtagatgctgaagaaatgacagctgttatcagttgtaggaatatccaaggaaacctctggaacaattccctggttatacctcgttcacgtcctccgtgaatgtaatggcgccatgcaactcgaggggatgccactgtcctcaatcaacagatcccagcctggataaggtcacaatggctcctttgaggccaaggctgtacactcgacgaccttggctggatccccgtggtgcccatagacaagcgcccggacccgggcaggctcggcggatgcggagtaggaggaggcggcaggtccgtgacagccagaagctgggagcagcccccgccactgccgggcgggggttcgcacccgccacagggtactgcagacccacatgctcgctccaaccaacacagagcctgac

SEQ ID NO: 11041 - RNA, 2096 nt, Homo sapiens
  source 1..2096: mol_type = other RNA
ctgaatagctgggactacaggtgcacagcaccatacctggctaatgtttgtattttttgtagagatggtgtttcaccacgttacctaggttgaccttgaactcctgggctcaagtgatccgcttgccttggcttcccaaagtgctgggattacaggtgtgagccaccgcgccaggccttgggtaattctttgttgcagtagactgttctgtgtcctgtggtgggtttaacagcagcactcactctgcctgctagatgccagtagcaacctccttcataagctgtgatagccagaaatatccccagacattgtcaaatgtctcctgggggtaaaattgcctctggttgagaaccactggtatattgtctatgtctccagttagaagggcagttccatgagagtgaagaccccacgtccaagttcctcagggccctgatgacctcagcctggcattcactcttccatgcagctgatcctccccaagccctggactgggccgcaggctacctgagaagcacatcaaagcgtttgttctacaggaccctcgtctgtgggcttgtgcagcttggggccagggatggtggcctactggcctttgcactgccagtacccacccaggctttgctttcagggtggtcagaaaatgattactgggggaacacatgacagaaaagcaggaagggggcctcttggtgctgtgagctgaccagtgcacagtgttggtccttctcgacagggatgacttctactttttggaagggagagttcagactttattagataccttaaggctggccctggggaaaaccgtggctggcttcaccatcctcctaataggaagaggcagtgaggagaacagtagtctggggaaggtgggagccccaactgaggggcctgcacccagcccctcagatccgcctcccctcccatgtcactccagctcttttgggatgatcacatggtgagaatctgctttgaagatatgaagggcttcatggaggcttccaaggcagactggtagtcctgcagcgggacctgggagcaggcaggggctgtgagctggcctcggcggatgagatcgcacagtgtgaggatcagctccttgaactggtctggactgtgatccttcttccactgggacaaccaaaagcctcgaagtttgagatccttaaaaatgagcaggctcacagaggctacgacgggctgcttggccatccccccataggttaccatggttcctccacgcgctaactgccgcagcagctctgtggagcttttcccaccaacacagttgagagcaagccgtggctggggcatgtccttaaagaagtttttcatttcgggccttcttagctcctcttctgtgatgacatgctcagcccccagactcttcagtctgtcactcagcttctggatatcaggtctgtctcggaccacattgatggttcttaggcccagggctgcggcgatctggatgactgcttgccccactccgctgttggatgcattctggatgacagaatcccctggctgcagttgctcgaagtccatcaacatcctgtaggctgtgcagggattgacacccagggtggcagcgctctgaagagggatgtcactcggaacttggatcagtgcttcctcgctgaacacagcctcggtccgccaggttcctaaaccagcatttgctggaatcacccagtctcctggcttcagcccggtcacattgctgcccaccgctaccacctgtgcaacaccttcgttccctccaacagcaggcagttcaggaaggaatccgtagtttccttggatcatatttatgtcagatggattgataggggccgccagcatcttcacacggacatctgatcctctcacagcagctagctccaggttcttgagtcttggctggatccccgtggtgcccatagacaagcgcccggacccgggcaggctcggcggatgcggagtaggaggaggcggcaggtccgtgacagccagaagctgggagcagcccccgccactgccgggcgggggttcgcacccgccacagggtactgcagacccacatgctcgctccaaccaacacagagcctgac

SEQ ID NO: 11042 - RNA, 2104 nt, Homo sapiens
  source 1..2104: mol_type = other RNA
ctgaatagctgggactacaggtgcacagcaccatacctggctaatgtttgtattttttgtagagatggtgtttcaccacgttacctaggttgaccttgaactcctgggctcaagtgatccgcttgccttggcttcccaaagtgctgggattacaggtgtgagccaccgcgccaggccttgggtaattctttgttgcagtagactgttctgtgtcctgtggtgggtttaacagcagcactcactctgcctgctagatgccagtagcaacctccttcataagctgtgatagccagaaatatccccagacattgtcaaatgtctcctgggggtaaaattgcctctggttgagaaccactggtatattgtctatgtctccagttagaagggcagttccatgagagtgaagaccccacgtccaagttcctcagggccctgatgacctcagcctggcattcactcttccatgcagctgatcctccccaagccctggactgggccgcaggctacctgagaagcacatcaaagcgtttgttctacaggaccctcgtctgtgggcttgtgcagcttggggccagggatggtggcctactggcctttgcactgccagtacccacccaggctttgctttcagggtggtcagaaaatgattactgggggaacacatgacagaaaagcaggaagggggcctcttggtgctgtgagctgaccagtgcacagtgttggtccttctcgacagggatgacttctactttttggaagggagagttcagactttattagataccttaaggctggccctggggaaaaccgtggctggcttcaccatcctcctaataggaagaggcagtgaggagaacagtagtctggggaaggtgggagccccaactgaggggcctgcacccagcccctcagatccgcctcccctcccatgtcactccagctcttttgggatgatcacatggtgagaatctgctttgaagatatgaagggcttcatggaggcttccaaggcagactggtagtcctgcagcgggacctgggagcaggcaggggctgtgagctggcctcggcggatgagatcgcacagtgtgaggatcagctccttgaactggtctggactgtgatccttcttccactgggacaaccaaaagcctcgaagtttgagatccttaaaaatgagcaggctcacagaggctacgacgggctgcttggccatccccccataggttaccatggttcctccacgcgctaactgccgcagcagctctgtggagcttttcccaccaacacagttgagagcaagccgtggctggggcatgtccttaaagaagtttttcatttcgggccttcttagctcctcttctgtgatgacatgctcagcccccagactcttcagtctgtcactcagcttctggatatcaggtctgtctcggaccacattgatggttcttaggcccagggctgcggcgatctggatgactgcttgccccactccgctgttggatgcattctggatgacagaatcccctggctgcagttgctcgaagtccatcaacatcctgtaggctgtgcagggattgacacccagggtggcagcgctctgaagagggatgtcactcggaacttggatcagtgcttcctcgctgaacacagcctcggtccgccaggttcctaaaccagcatttgctggaatcacccagtctcctggcttcagcccggtcacattgctgcccaccgctaccacctgtgcaacaccttcgttccctccaacagcaggcagttcaggaaggaatccgtagtttccttggatcatatttatgtcagatggattgataggggccgccagcatcttcacacggacatctgatcctctcacagcagctagctccaggttcttgagttcgacgaccttggctggatccccgtggtgcccatagacaagcgcccggacccgggcaggctcggcggatgcggagtaggaggaggcggcaggtccgtgacagccagaagctgggagcagcccccgccactgccgggcgggggttcgcacccgccacagggtactgcagacccacatgctcgctccaaccaacacagagcctgac

SEQ ID NO: 11043 - RNA, 2357 nt, Homo sapiens
  source 1..2357: mol_type = other RNA
ctgaatagctgggactacaggtgcacagcaccatacctggctaatgtttgtattttttgtagagatggtgtttcaccacgttacctaggttgaccttgaactcctgggctcaagtgatccgcttgccttggcttcccaaagtgctgggattacaggtgtgagccaccgcgccaggccttgggtaattctttgttgcagtagactgttctgtgtcctgtggtgggtttaacagcagcactcactctgcctgctagatgccagtagcaacctccttcataagctgtgatagccagaaatatccccagacattgtcaaatgtctcctgggggtaaaattgcctctggttgagaaccactggtatattgtctatgtctccagttagaagggcagttccatgagagtgaagaccccacgtccaagttcctcagggccctgatgacctcagcctggcattcactcttccatgcagctgatcctccccaagccctggactgggccgcaggctacctgagaagcacatcaaagcgtttgttctacaggaccctcgtctgtgggcttgtgcagcttggggccagggatggtggcctactggcctttgcactgccagtacccacccaggctttgctttcagggtggtcagaaaatgattactgggggaacacatgacagaaaagcaggaagggggcctcttggtgctgtgagctgaccagtgcacagtgttggtccttctcgacagggatgacttctactttttggaagggagagttcagactttattagataccttaaggctggccctggggaaaaccgtggctggcttcaccatcctcctaataggaagaggcagtgaggagaacagtagtctggggaaggtgggagccccaactgaggggcctgcacccagcccctcagatccgcctcccctcccatgtcactccagctcttttgggatgatcacatggtgagaatctgctttgaagatatgaagggcttcatggaggcttccaaggcagactggtagtcctgcagcgggacctgggagcaggcaggggctgtgagctggcctcggcggatgagatcgcacagtgtgaggatcagctccttgaactggtctggactgtgatccttcttccactgggacaaccaaaagcctcgaagtttgagatccttaaaaatgagcaggctcacagaggctacgacgggctgcttggccatccccccataggttaccatggttcctccacgcgctaactgccgcagcagctctgtggagcttttcccaccaacacagttgagagcaagccgtggctggggcatgtctaggcatgttgtggggtggaggttctggaaggttaagaggctttgagttcggagagactgaggccagctctgactctctggagcccttataaactatatgattttggttaagcatttcctcttttctgagtcttagtttcctaatcttaaagaagtttttcatttcgggccttcttagctcctcttctgtgatgacatgctcagcccccagactcttcagtctgtcactcagcttctggatatcaggtctggctgcagttgctcgaagtccatcaacatcctgtaggctgtgcagggattgacacccagggtggcagcgctctgaagagggatgtcactcggaacttggatcagtgcttcctcgctgaacacagcctcggtccgccaggttcctaaaccagcatttgctggaatcacccagtctcctggcttcagcccggtcacattgctgcccaccgctaccacctgtgcaacaccttcgttccctccaacagcaggcagttcaggaaggaatccgtagtttccttggatcatatttatgtcagatggattgataggggccgccagcatcttcacacggacatctgatcctctcacagcagctagctccaggttcttgagtctaagcacaaagccaaacggagatgttcatgtcatccaggctagaatgggtgtttcgctcaaatcatctcctcaaagtaggtcaggcaacatttctgagctgccatgtgtgcccaggaattacggttacagtagatgctgaagaaatgacagctgttatcagttgtaggaatatccaaggaaacctctggaacaattccctggttataccttcgacgaccttggctggatccccgtggtgcccatagacaagcgcccggacccgggcaggctcggcggatgcggagtaggaggaggcggcaggtccgtgacagccagaagctgggagcagcccccgccactgccgggcgggggttcgcacccgccacagggtactgcagacccacatgctcgctccaaccaacacagagcctgac

SEQ ID NO: 11044 - RNA, 1954 nt, Homo sapiens
  source 1..1954: mol_type = other RNA
ctgaatagctgggactacaggtgcacagcaccatacctggctaatgtttgtattttttgtagagatggtgtttcaccacgttacctaggttgaccttgaactcctgggctcaagtgatccgcttgccttggcttcccaaagtgctgggattacaggtgtgagccaccgcgccaggccttgggtaattctttgttgcagtagactgttctgtgtcctgtggtgggtttaacagcagcactcactctgcctgctagatgccagtagcaacctccttcataagctgtgatagccagaaatatccccagacattgtcaaatgtctcctgggggtaaaattgcctctggttgagaaccactggtatattgtctatgtctccagttagaagggcagttccatgagagtgaagaccccacgtccaagttcctcagggccctgatgacctcagcctggcattcactcttccatgcagctgatcctccccaagccctggactgggccgcaggctaccttaaggctggccctggggaaaaccgtggctggcttcaccatcctcctaataggaagaggcagtgaggagaacagtagtctggggaaggtgggagccccaactgaggggcctgcacccagcccctcagatccgcctcccctcccatgtcactccagctcttttgggatgatcacatggtgagaatctgctttgaagatatgaagggcttcatggaggcttccaaggcagactggtagtcctgcagcgggacctgggagcaggcaggggctgtgagctggcctcggcggatgagatcgcacagtgtgaggatcagctccttgaactggtctggactgtgatccttcttccactgggacaaccaaaagcctcgaagtttgagatccttaaaaatgagcaggctcacagaggctacgacgggctgcttggccatccccccataggttaccatggttcctccacgcgctaactgccgcagcagctctgtggagcttttcccaccaacacagttgagagcaagccgtggctggggcatgtccttaaagaagtttttcatttcgggccttcttagctcctcttctgtgatgacatgctcagcccccagactcttcagtctgtcactcagcttctggatatcaggtctgtctcggaccacattgatggttcttaggcccagggctgcggcgatctggatgactgcttgccccactccgctgttggatgcattctggatgacagaatcccctggctgcagttgctcgaagtccatcaacatcctgtaggctgtgcagggattgacacccagggtggcagcgctctgaagagggatgtcactcggaacttggatcagtgcttcctcgctgaacacagcctcggtccgccaggttcctaaaccagcatttgctggaatcacccagtctcctggcttcagcccggtcacattgctgcccaccgctaccacctgtgcaacaccttcgttccctccaacagcaggcagttcaggaaggaatccgtagtttccttggatcatatttatgtcagatggattgataggggccgccagcatcttcacacggacatctgatcctctcacagcagctagctccaggttcttgagtctaagcacaaagccaaacggagatgttcatgtcatccaggctagaatgggtgtttcgctcaaatcatctcctcaaagtaggtcaggcaacatttctgagctgccatgtgtgcccaggaattacggtttcgacgaccttggctggatccccgtggtgcccatagacaagcgcccggacccgggcaggctcggcggatgcggagtaggaggaggcggcaggtccgtgacagccagaagctgggagcagcccccgccactgccgggcgggggttcgcacccgccacagggtactgcagacccacatgctcgctccaaccaacacagagcctgac

SEQ ID NO: 11045 - RNA, 1827 nt, Homo sapiens
  source 1..1827: mol_type = other RNA
ctgaatagctgggactacaggtgcacagcaccatacctggctaatgtttgtattttttgtagagatggtgtttcaccacgttacctaggttgaccttgaactcctgggctcaagtgatccgcttgccttggcttcccaaagtgctgggattacaggtgtgagccaccgcgccaggccttgggtaattctttgttgcagtagactgttctgtgtcctgtggtgggtttaacagcagcactcactctgcctgctagatgccagtagcaacctccttcataagctgtgatagccagaaatatccccagacattgtcaaatgtctcctgggggtaaaattgcctctggttgagaaccactggtatattgtctatgtctccagttagaagggcagttccatgagagtgaagaccccacgtccaagttcctcagggccctgatgacctcagcctggcattcactcttccatgcagctgatcctccccaagccctggactgggccgcaggctaccttaaggctggccctggggaaaaccgtggctggcttcaccatcctcctaataggaagaggcagtgaggagaacagtagtctggggaaggtgggagccccaactgaggggcctgcacccagcccctcagatccgcctcccctcccatgtcactccagctcttttgggatgatcacatggtgagaatctgctttgaagatatgaagggcttcatggaggcttccaaggcagactggtagtcctgcagcgggacctgggagcaggcaggggctgtgagctggcctcggcggatgagatcgcacagtgtgaggatcagctccttgaactggtctggactgtgatccttcttccactgggacaaccaaaagcctcgaagtttgagatccttaaaaatgagcaggctcacagaggctacgacgggctgcttggccatccccccataggttaccatggttcctccacgcgctaactgccgcagcagctctgtggagcttttcccaccaacacagttgagagcaagccgtggctggggcatgtccttaaagaagtttttcatttcgggccttcttagctcctcttctgtgatgacatgctcagcccccagactcttcagtctgtcactcagcttctggatatcaggtctgtctcggaccacattgatggttcttaggcccagggctgcggcgatctggatgactgcttgccccactccgctgttggatgcattctggatgacagaatcccctggctgcagttgctcgaagtccatcaacatcctgtaggctgtgcagggattgacacccagggtggcagcgctctgaagagggatgtcactcggaacttggatcagtgcttcctcgctgaacacagcctcggtccgccaggttcctaaaccagcatttgctggaatcacccagtctcctggcttcagcccggtcacattgctgcccaccgctaccacctgtgcaacaccttcgttccctccaacagcaggcagttcaggaaggaatccgtagtttccttggatcatatttatgtcagatggattgataggggccgccagcatcttcacacggacatctgatcctctcacagcagctagctccaggttcttgagttcgacgaccttggctggatccccgtggtgcccatagacaagcgcccggacccgggcaggctcggcggatgcggagtaggaggaggcggcaggtccgtgacagccagaagctgggagcagcccccgccactgccgggcgggggttcgcacccgccacagggtactgcagacccacatgctcgctccaaccaacacagagcctgac

SEQ ID NO: 11046 - RNA, 6291 nt, Homo sapiens
  source 1..6291: mol_type = other RNA
ctgaatagctgggactacaggtgcacatcaccacatccaggtaattattttactttttgaatcatgatatgtagcaaccaatctgggaattatttattcataaaagataacattttcctgctaactccaacctcagaaaaaatgtattatgcctgactcaaatatgtcattatttttatgagaaaaagagtcatattgaagtaattatgtctatatgtaataattatcattatttgagataatttgcattggggagaaaagcaggcaatcagaaattacatattcaaggctgggcgcagtggctcacgcctgtaatcccagcactttgggaggcagaggcgagtgaatcacctgaggtcagagttcaagaccagcctgaccaacaaggagaaaccccatctctactaaaacaaaacaaaacaaaacaaaacaaaaaaagccacaaaattagccgggcatggtggcacatgcctgtaattccagttactcgggaggctgaggcaggagaattgcttgaacctgggaggcagaggttgtagtaagccgagattgtgccactgcacgccagcctgggcgacaagaacgagactcagtctcaaaaaaaaaaaaaaagaaagaaagaaagaaattacatattcaggttctagcaaatgcagttctctaataaacactaaataaatcataatacaagttacagttaaacctaattgttttactatataggatgtatcttttttgtacctatattttatcttcctttgcttctctggcctctattgggaggcagcacggtagtgaacacctcggggatctttctggttacgtaaacctgagttttaattttggttcatactaccttttaactttgggtagtctgctgagcttgttttttgttttcactcatctgtcatatcaagctagtaataattctgccatggttttggttttcatattgaaaggcattacataagcaaaatgcataacatataaatattagttccctttccactatgcatccaatctccctattaaattaagcctaaaaataataatttttgttttattaaaagccttccacattctacatatgaaagggattttttaaaggtgttttagataaaaaatgtttcaaccaactgaccaagaatatctcttcatatttatgtcatctacataaaaacttacatttatatcatatatcttttagtcttcttttctatattcttgattgtcatgttgtacagccagaaaagaatgagtataaattatctagattttttaaagtgcacattcaaacatagaaaatctaattattttacttgtttcttagtattaggctgaggccaatgagtccatgagctaaagggttgaaacttggcaccaaaaaagtgattgtttatgagtcctgtagatttatactgagaaaacatcatgtcttccaatgtgaaatacactaaaacctgattttttgtctcttaaggtgtgctaggtgaatgcaaaaaggatcaggaaagggggtgaggataggtcaggaaaagtgcaaacacaatgttctattcataaattagtgatggcatatttaaggttaagtagtaaaaaatatggggggctcagttaacacgaatgaaaaaatagttaaagtagccatgaattatctggataccttgatttaatgacaccctttcttctgtacaatttcataatgtgggaatagagattagtggggattgtagtggtataccctgactttgcttcatgatatctcaaatgtttaaaacctattattccctagagaaagaaatatgttcatactaattgttgcagaggcagaagccaaatatatctcctcctccatttatgtgactatatagtaatgaaaatcctaggttgatacacttttctcaatcttggaaagattctgctaaagcagcaaatcttctaacaagttcaagagggtggggagagtgaacaagtagaataatttatattaccctggaacaattctgaatcctgtaggtatttatgtcactgtttcaattgtgttctggtttaactgtcaatatttatgcatagcagttaacgtgtgtgcatatttgtaactgtgcagtgctactgccaggtgtgactgtacaaatcatgtgctttgaatgtgcaagttttactttcttttctaacaatttaatacagtgttagaaataaataacgaatgaagacaaccaaagagcagccagacaaatgtgaactggttttgacgtgacgagaaactcatcagtaagtaaataaacctcctccctggagaaggccactgaaatgcacccaggaggatgtctctactagaaggtaataaaaaatatatataatgtagtctttgacctaaaacctcatgattattactttgccatttatttccccctggtatctgatgttcatattagtttaatgtgccttttcagagaattcaagacactttttggaaagtagaatttttttttgaaaatttatgattggagaggtactacacaatttagaggttacatttcttgacaaatctgagttgaataaaaaagaactaaaaatataaacatagctaattcaagaatcaagatcgggtgaaactaaattaaaaacagccataaagtcccacattttccctaatttatttacctatgatattggcacatcttgttttacttaacatttgaaaaatacaaatatctcttcatatgcaaaagagcaaatgttaaatgaaaaactgaattttatatagcttcctaaatatgagccacatgcttaagcagtgaattaactttatgaatcaaatgtttaatgttaactattacaaaagcctggtatccaggtgcaatctcaccagaaaaaaatagcacctgcctttattacaataaaaaaaatggctaattccctttgacatcttaagagtgacactactttgtcaagcactaaatactttttaaattaatcatgttaaacttcagatttatagatataaatattgtatttataactttagtcataatgtacaatttctttcttgtttaaaagtactttctcactcaaaatggtatttatagtttaaaaagaatatgcctctgtattcaggagtgattcaaattcccagatgttttcacatagttatgaaaatgggaaagtgctgaattaaactgggctgcaatatttcaagttttttgctatcaggttataaactatacctacgattgcaagtcatacagtgcctctatttctagaaggcttttaaagtttcctggcttagttatgtccaaaggcagcaggaagtctcatcagtagagggcagaattttcaagtgctgccattcttatcccaggaggcatttccagtggttgagcacaaggcctgtttgtagtttgcttttgctcttgcattttgtggaagggaaggaactgagagagcttagagggttcattaaaaccacccctcactctcttagtcgtagtcagatggagtattcataacagtaacctccaattaccactatgtgttgggaaaaattagaattcggtctacttacaatcctgccaactaggattttactttgatatttcagtataacagtgaatctggattgatgcctgattaaaataaaatccctgattattactttctggattacgaactaaaatccctgtaaaatcaatggatgtgactcattgttaagagtcatgcagacttttacatattaggtaagaattctaaaaattatttgagggttctattctctagcaccaggtactaatgctccctactcaaaaaaaatcatgtgcatggattaatcaagtctaacagtgctcagatttaatggtttaacattgattttcttttctttgtcaaacttatatatgcaaatatttttatagtagtcagatgttatttttgaataaggatcaccctcatttttacccatgtgcttatctttaaaaccaacattgtaaagtagcacgcagacatatgtttcttttatcttcatggattatttttaccttaaaaataaattatcatttttttttttgaatttgggttttattctccagatactctgtgtacatgtgggtaagtatgtgggagtatgtgtgtttgtgtgtaagaggggataattaattgtctctcaactctatctcatactttaatatcaaataaaaaatgaaatgtataaagggtcactttgtaggattaggcatcctccttctacctacttaaaccaggggtttgggattcagaattctccatataaccaagaccgaaagtcactggaagactttaaaattagtattttaaccaccacacccagagtcaggtatggaaataaacctatagcatggattctttctatgcataatctcaaaatttaactacccaaataagtaagtttttaaaaactaatttaaaatttgccattgaggaaaatatcacctccatccttaattgtgactcctcatttcagctaaaaccttttctaatactttaaaaaaacaaaatgaaaaacaaactcctagataaagtcataaacactgaaatcagagatgtgattcttgttaaatgttagtttctctttctgaggttacactctgtgcatttgaaactttgacgttaacatcttccgaatgtttagatttgctcaagggttcagattctctggtcttctgccttgcattttcctccttcctttcctttgcaagcaatctatagttgatagcattgccaatgagcagccacacgcttgctgctaccacaatagccccacaggacatgtacatgtatttatattctccagttaaatccaccaatttacctgcaagaggagggccaagaagaactgggccacactccacaattgtgacaagtccgacggcactggaaaatcttggtgcacccacgaggtccatgagagtttcaaagagaacactgctaacactcccaaatccaaggccaaaaaatacagcatataataccaggcttgtgtagtcctgtgccagtgggcacaagaggtgacacactccattgaacatgattgcaaaactgaagaagtactgaattcgaggtcgaatatatttggagtttgcaattaatcctacagaaggcctagcaaacatatcaacgaaagccataacagatagcagaaaagctgccgagtactcatcaattccttggtctttagcatatggagccaagaatataatgggggcaaaaaaacctaggaacataatgacatttccagacagatatatcagaaatcctctatgcttaaaaagggagaaatctaaatacttattaactttttcccaagttgatttcttcgttttgattttctttgggcttgaatcatcttctgttttgccagtcttatttttagacttagaagtggtttgattgggtccaaggggtctcatgagggaaccagccacacaggcattcaaaagtagacttcccaaaatcaggaagcttcctttccagccaaaagtattaaaaaggtactgattgaaaggagccaatgaacttaagaaaacaggacttcctgccatggccaatccatttgccatgggtcgcttcctatagaagtatttgccaattatggttaaggcgggttgcaggttgaaggctaaacctaaacctgtaatgaatcccatagtgaggtacagctgtaccacgctgctactaaaggaggccaacaccattccaagacagcataataagcctcctgctatcaccaccggccggctgccgtatttattcaccaaaacactacttacaggacctaggcatgatcctgattgagtaaagctgcactgaatcctcaaggatgtgaagatcaaaaagctttcaaatattctacctcaagtagatggtgatctctttaaagggtgaatgatgcattccgcttctccttttttcctcctgcgtacataacagccagcataatggatgaaatccatgctatttcactgtaggtagtgtggaatatttgctgaatttctttgaagaatacggtgacagctttggggaatgcataggaaaatccaatggagataaaagctgctccaaccacaatccaaccccatcctccatctggaggtggatgcacaggtggggcacttggcattggtggcatttctgctcctctagtggaaattcaagtaacctggcgacaggtgtttagaaacatggtcttccatttcaccaagacataagtttccctgatctatggactcctctccccacctgaggcagaagtttccttgt

SEQ ID NO: 11047 - RNA, 6533 nt, Homo sapiens
  source 1..6533: mol_type = other RNA
ctgaatagctgggactacaggtgcacatcaccacatccaggtaattattttactttttgaatcatgatatgtagcaaccaatctgggaattatttattcataaaagataacattttcctgctaactccaacctcagaaaaaatgtattatgcctgactcaaatatgtcattatttttatgagaaaaagagtcatattgaagtaattatgtctatatgtaataattatcattatttgagataatttgcattggggagaaaagcaggcaatcagaaattacatattcaaggctgggcgcagtggctcacgcctgtaatcccagcactttgggaggcagaggcgagtgaatcacctgaggtcagagttcaagaccagcctgaccaacaaggagaaaccccatctctactaaaacaaaacaaaacaaaacaaaacaaaaaaagccacaaaattagccgggcatggtggcacatgcctgtaattccagttactcgggaggctgaggcaggagaattgcttgaacctgggaggcagaggttgtagtaagccgagattgtgccactgcacgccagcctgggcgacaagaacgagactcagtctcaaaaaaaaaaaaaaagaaagaaagaaagaaattacatattcaggttctagcaaatgcagttctctaataaacactaaataaatcataatacaagttacagttaaacctaattgttttactatataggatgtatcttttttgtacctatattttatcttcctttgcttctctggcctctattgggaggcagcacggtagtgaacacctcggggatctttctggttacgtaaacctgagttttaattttggttcatactaccttttaactttgggtagtctgctgagcttgttttttgttttcactcatctgtcatatcaagctagtaataattctgccatggttttggttttcatattgaaaggcattacataagcaaaatgcataacatataaatattagttccctttccactatgcatccaatctccctattaaattaagcctaaaaataataatttttgttttattaaaagccttccacattctacatatgaaagggattttttaaaggtgttttagataaaaaatgtttcaaccaactgaccaagaatatctcttcatatttatgtcatctacataaaaacttacatttatatcatatatcttttagtcttcttttctatattcttgattgtcatgttgtacagccagaaaagaatgagtataaattatctagattttttaaagtgcacattcaaacatagaaaatctaattattttacttgtttcttagtattaggctgaggccaatgagtccatgagctaaagggttgaaacttggcaccaaaaaagtgattgtttatgagtcctgtagatttatactgagaaaacatcatgtcttccaatgtgaaatacactaaaacctgattttttgtctcttaaggtgtgctaggtgaatgcaaaaaggatcaggaaagggggtgaggataggtcaggaaaagtgcaaacacaatgttctattcataaattagtgatggcatatttaaggttaagtagtaaaaaatatggggggctcagttaacacgaatgaaaaaatagttaaagtagccatgaattatctggataccttgatttaatgacaccctttcttctgtacaatttcataatgtgggaatagagattagtggggattgtagtggtataccctgactttgcttcatgatatctcaaatgtttaaaacctattattccctagagaaagaaatatgttcatactaattgttgcagaggcagaagccaaatatatctcctcctccatttatgtgactatatagtaatgaaaatcctaggttgatacacttttctcaatcttggaaagattctgctaaagcagcaaatcttctaacaagttcaagagggtggggagagtgaacaagtagaataatttatattaccctggaacaattctgaatcctgtaggtatttatgtcactgtttcaattgtgttctggtttaactgtcaatatttatgcatagcagttaacgtgtgtgcatatttgtaactgtgcagtgctactgccaggtgtgactgtacaaatcatgtgctttgaatgtgcaagttttactttcttttctaacaatttaatacagtgttagaaataaataacgaatgaagacaaccaaagagcagccagacaaatgtgaactggttttgacgtgacgagaaactcatcagtaagtaaataaacctcctccctggagaaggccactgaaatgcacccaggaggatgtctctactagaaggtaataaaaaatatatataatgtagtctttgacctaaaacctcatgattattactttgccatttatttccccctggtatctgatgttcatattagtttaatgtgccttttcagagaattcaagacactttttggaaagtagaatttttttttgaaaatttatgattggagaggtactacacaatttagaggttacatttcttgacaaatctgagttgaataaaaaagaactaaaaatataaacatagctaattcaagaatcaagatcgggtgaaactaaattaaaaacagccataaagtcccacattttccctaatttatttacctatgatattggcacatcttgttttacttaacatttgaaaaatacaaatatctcttcatatgcaaaagagcaaatgttaaatgaaaaactgaattttatatagcttcctaaatatgagccacatgcttaagcagtgaattaactttatgaatcaaatgtttaatgttaactattacaaaagcctggtatccaggtgcaatctcaccagaaaaaaatagcacctgcctttattacaataaaaaaaatggctaattccctttgacatcttaagagtgacactactttgtcaagcactaaatactttttaaattaatcatgttaaacttcagatttatagatataaatattgtatttataactttagtcataatgtacaatttctttcttgtttaaaagtactttctcactcaaaatggtatttatagtttaaaaagaatatgcctctgtattcaggagtgattcaaattcccagatgttttcacatagttatgaaaatgggaaagtgctgaattaaactgggctgcaatatttcaagttttttgctatcaggttataaactatacctacgattgcaagtcatacagtgcctctatttctagaaggcttttaaagtttcctggcttagttatgtccaaaggcagcaggaagtctcatcagtagagggcagaattttcaagtgctgccattcttatcccaggaggcatttccagtggttgagcacaaggcctgtttgtagtttgcttttgctcttgcattttgtggaagggaaggaactgagagagcttagagggttcattaaaaccacccctcactctcttagtcgtagtcagatggagtattcataacagtaacctccaattaccactatgtgttgggaaaaattagaattcggtctacttacaatcctgccaactaggattttactttgatatttcagtataacagtgaatctggattgatgcctgattaaaataaaatccctgattattactttctggattacgaactaaaatccctgtaaaatcaatggatgtgactcattgttaagagtcatgcagacttttacatattaggtaagaattctaaaaattatttgagggttctattctctagcaccaggtactaatgctccctactcaaaaaaaatcatgtgcatggattaatcaagtctaacagtgctcagatttaatggtttaacattgattttcttttctttgtcaaacttatatatgcaaatatttttatagtagtcagatgttatttttgaataaggatcaccctcatttttacccatgtgcttatctttaaaaccaacattgtaaagtagcacgcagacatatgtttcttttatcttcatggattatttttaccttaaaaataaattatcatttttttttttgaatttgggttttattctccagatactctgtgtacatgtgggtaagtatgtgggagtatgtgtgtttgtgtgtaagaggggataattaattgtctctcaactctatctcatactttaatatcaaataaaaaatgaaatgtataaagggtcactttgtaggattaggcatcctccttctacctacttaaaccaggggtttgggattcagaattctccatataaccaagaccgaaagtcactggaagactttaaaattagtattttaaccaccacacccagagtcaggtatggaaataaacctatagcatggattctttctatgcataatctcaaaatttaactacccaaataagtaagtttttaaaaactaatttaaaatttgccattgaggaaaatatcacctccatccttaattgtgactcctcatttcagctaaaaccttttctaatactttaaaaaaacaaaatgaaaaacaaactcctagataaagtcataaacactgaaatcagagatgtgattcttgttaaatgttagtttctctttctgaggttacactctgtgcatttgaaactttgacgttaacatcttccgaatgtttagatttgctcaagggttcagattctctggtcttctgccttgcattttcctccttcctttcctttgcaagcaatctatagttgatagcattgccaatgagcagccacacgcttgctgctaccacaatagccccacaggacatgtacatgtatttatattctccagttaaatccaccaatttacctgcaagaggagggccaagaagaactgggccacactccacaattgtgacaagtccgacggcactggaaaatcttggtgcacccacgaggtccatgagagtttcaaagagaacactgctaacactcccaaatccaaggccaaaaaatacagcatataataccaggcttgtgtagtcctgtgccagtgggcacaagaggtgacacactccattgaacatgattgcaaaactgaagaagtactgaattcgaggtcgaatatatttggagtttgcaattaatcctacagaaggcctagcaaacatatcaacgaaagccataacagatagcagaaaagctgccgagtactcatcaattccttggtctttagcatatggagccaagaatataatgggggcaaaaaaacctaggaacataatgacatttccagacagatatatcagaaatcctctatgcttaaaaagggagaaatctaaatacttattaactttttcccaagttgatttcttcgttttgattttctttgggcttgaatcatcttctgttttgccagtcttatttttagacttagaagtggtttgattgggtccaaggggtctcatgagggaaccagccacacaggcattcaaaagtagacttcccaaaatcaggaagcttcctttccagccaaaagtattaaaaaggtactgattgaaaggagccaatgaacttaagaaaacaggacttcctgccatggccaatccatttgccatgggtcgcttcctatagaagtatttgccaattatggttaaggcgggttgcaggttgaaggctaaacctaaacctgtaatgaatcccatagtgaggtacagctgtaccacgctgctactaaaggaggccaacaccattccaagacagcataataagcctcctgctatcaccaccggccggctgccgtatttattcaccaaaacactacttacaggacctaggcatgatcctgattgagtaaagctgcactgaatcctcaaggatgtgaagatcaaaaagctttcaaatattctacctcctgcgtacataacagccagcataatggatgaaatccatgctatttcactgtaggtagtgtggaatatttgctgaatttctttgaagaatacggtgacagctttggggaatgcataggaaaatccaatggagataaaagctgctccaaccacaatccaaccccatcctccatctggaggtggatgcacaggtggggcacttggcattggtggcatttctgctcctctagtggaaattcaagtaacagagtaactctgttggcaccaagagtcccagagtctttggttccccagatcaccttgtttcaggtttcacaggaaagtatcacatcttaagattgactctttatctggtctctggcgcagggtgggcgctgcagccctccgttcccagcaaaccgcagccgattcgcctcgctgtcaacgggtgaatggaattatttatttatttatggcccctgacgtgtcctcgcccgccacagccagcggagaaggaggcggtggcgggaaggggaggcgcggctgctgaacgcccttgtgggtgcggaggagcgcgcgccaggggtgggggccggacaggctgcggtggaggccggcccggggggtggtgggggggagccgcctcccggtgcctggagaccgactgag

SEQ ID NO: 11048 - RNA, 7158 nt, Homo sapiens
  source 1..7158: mol_type = other RNA
ctgaatagctgggactacaggtgcacatcaccacatccaggtaattattttactttttgaatcatgatatgtagcaaccaatctgggaattatttattcataaaagataacattttcctgctaactccaacctcagaaaaaatgtattatgcctgactcaaatatgtcattatttttatgagaaaaagagtcatattgaagtaattatgtctatatgtaataattatcattatttgagataatttgcattggggagaaaagcaggcaatcagaaattacatattcaaggctgggcgcagtggctcacgcctgtaatcccagcactttgggaggcagaggcgagtgaatcacctgaggtcagagttcaagaccagcctgaccaacaaggagaaaccccatctctactaaaacaaaacaaaacaaaacaaaacaaaaaaagccacaaaattagccgggcatggtggcacatgcctgtaattccagttactcgggaggctgaggcaggagaattgcttgaacctgggaggcagaggttgtagtaagccgagattgtgccactgcacgccagcctgggcgacaagaacgagactcagtctcaaaaaaaaaaaaaaagaaagaaagaaagaaattacatattcaggttctagcaaatgcagttctctaataaacactaaataaatcataatacaagttacagttaaacctaattgttttactatataggatgtatcttttttgtacctatattttatcttcctttgcttctctggcctctattgggaggcagcacggtagtgaacacctcggggatctttctggttacgtaaacctgagttttaattttggttcatactaccttttaactttgggtagtctgctgagcttgttttttgttttcactcatctgtcatatcaagctagtaataattctgccatggttttggttttcatattgaaaggcattacataagcaaaatgcataacatataaatattagttccctttccactatgcatccaatctccctattaaattaagcctaaaaataataatttttgttttattaaaagccttccacattctacatatgaaagggattttttaaaggtgttttagataaaaaatgtttcaaccaactgaccaagaatatctcttcatatttatgtcatctacataaaaacttacatttatatcatatatcttttagtcttcttttctatattcttgattgtcatgttgtacagccagaaaagaatgagtataaattatctagattttttaaagtgcacattcaaacatagaaaatctaattattttacttgtttcttagtattaggctgaggccaatgagtccatgagctaaagggttgaaacttggcaccaaaaaagtgattgtttatgagtcctgtagatttatactgagaaaacatcatgtcttccaatgtgaaatacactaaaacctgattttttgtctcttaaggtgtgctaggtgaatgcaaaaaggatcaggaaagggggtgaggataggtcaggaaaagtgcaaacacaatgttctattcataaattagtgatggcatatttaaggttaagtagtaaaaaatatggggggctcagttaacacgaatgaaaaaatagttaaagtagccatgaattatctggataccttgatttaatgacaccctttcttctgtacaatttcataatgtgggaatagagattagtggggattgtagtggtataccctgactttgcttcatgatatctcaaatgtttaaaacctattattccctagagaaagaaatatgttcatactaattgttgcagaggcagaagccaaatatatctcctcctccatttatgtgactatatagtaatgaaaatcctaggttgatacacttttctcaatcttggaaagattctgctaaagcagcaaatcttctaacaagttcaagagggtggggagagtgaacaagtagaataatttatattaccctggaacaattctgaatcctgtaggtatttatgtcactgtttcaattgtgttctggtttaactgtcaatatttatgcatagcagttaacgtgtgtgcatatttgtaactgtgcagtgctactgccaggtgtgactgtacaaatcatgtgctttgaatgtgcaagttttactttcttttctaacaatttaatacagtgttagaaataaataacgaatgaagacaaccaaagagcagccagacaaatgtgaactggttttgacgtgacgagaaactcatcagtaagtaaataaacctcctccctggagaaggccactgaaatgcacccaggaggatgtctctactagaaggtaataaaaaatatatataatgtagtctttgacctaaaacctcatgattattactttgccatttatttccccctggtatctgatgttcatattagtttaatgtgccttttcagagaattcaagacactttttggaaagtagaatttttttttgaaaatttatgattggagaggtactacacaatttagaggttacatttcttgacaaatctgagttgaataaaaaagaactaaaaatataaacatagctaattcaagaatcaagatcgggtgaaactaaattaaaaacagccataaagtcccacattttccctaatttatttacctatgatattggcacatcttgttttacttaacatttgaaaaatacaaatatctcttcatatgcaaaagagcaaatgttaaatgaaaaactgaattttatatagcttcctaaatatgagccacatgcttaagcagtgaattaactttatgaatcaaatgtttaatgttaactattacaaaagcctggtatccaggtgcaatctcaccagaaaaaaatagcacctgcctttattacaataaaaaaaatggctaattccctttgacatcttaagagtgacactactttgtcaagcactaaatactttttaaattaatcatgttaaacttcagatttatagatataaatattgtatttataactttagtcataatgtacaatttctttcttgtttaaaagtactttctcactcaaaatggtatttatagtttaaaaagaatatgcctctgtattcaggagtgattcaaattcccagatgttttcacatagttatgaaaatgggaaagtgctgaattaaactgggctgcaatatttcaagttttttgctatcaggttataaactatacctacgattgcaagtcatacagtgcctctatttctagaaggcttttaaagtttcctggcttagttatgtccaaaggcagcaggaagtctcatcagtagagggcagaattttcaagtgctgccattcttatcccaggaggcatttccagtggttgagcacaaggcctgtttgtagtttgcttttgctcttgcattttgtggaagggaaggaactgagagagcttagagggttcattaaaaccacccctcactctcttagtcgtagtcagatggagtattcataacagtaacctccaattaccactatgtgttgggaaaaattagaattcggtctacttacaatcctgccaactaggattttactttgatatttcagtataacagtgaatctggattgatgcctgattaaaataaaatccctgattattactttctggattacgaactaaaatccctgtaaaatcaatggatgtgactcattgttaagagtcatgcagacttttacatattaggtaagaattctaaaaattatttgagggttctattctctagcaccaggtactaatgctccctactcaaaaaaaatcatgtgcatggattaatcaagtctaacagtgctcagatttaatggtttaacattgattttcttttctttgtcaaacttatatatgcaaatatttttatagtagtcagatgttatttttgaataaggatcaccctcatttttacccatgtgcttatctttaaaaccaacattgtaaagtagcacgcagacatatgtttcttttatcttcatggattatttttaccttaaaaataaattatcatttttttttttgaatttgggttttattctccagatactctgtgtacatgtgggtaagtatgtgggagtatgtgtgtttgtgtgtaagaggggataattaattgtctctcaactctatctcatactttaatatcaaataaaaaatgaaatgtataaagggtcactttgtaggattaggcatcctccttctacctacttaaaccaggggtttgggattcagaattctccatataaccaagaccgaaagtcactggaagactttaaaattagtattttaaccaccacacccagagtcaggtatggaaataaacctatagcatggattctttctatgcataatctcaaaatttaactacccaaataagtaagtttttaaaaactaatttaaaatttgccattgaggaaaatatcacctccatccttaattgtgactcctcatttcagctaaaaccttttctaatactttaaaaaaacaaaatgaaaaacaaactcctagataaagtcataaacactgaaatcagagatgtgattcttgttaaatgttagtttctctttctgaggttacactctgtgcatttgaaactttgacgttaacatcttccgaatgtttagatttgctcaagggttcagattctctggtcttctgccttgcattttcctccttcctttcctttgcaagcaatctatagttgatagcattgccaatgagcagccacacgcttgctgctaccacaatagccccacaggacatgtacatgtatttatattctccagttaaatccaccaatttacctgcaagaggagggccaagaagaactgggccacactccacaattgtgacaagtccgacggcactggaaaatcttggtgcacccacgaggtccatgagagtttcaaagagaacactgctaacactcccaaatccaaggccaaaaaatacagcatataataccaggcttgtgtagtcctgtgccagtgggcacaagaggtgacacactccattgaacatgattgcaaaactgaagaagtactgaattcgaggtcgaatatatttggagtttgcaattaatcctacagaaggcctagcaaacatatcaacgaaagccataacagatagcagaaaagctgccgagtactcatcaattccttggtctttagcatatggagccaagaatataatgggggcaaaaaaacctaggaacataatgacatttccagacagatatatcagaaatcctctatgcttaaaaagggagaaatctaaatacttattaactttttcccaagttgatttcttcgttttgattttctttgggcttgaatcatcttctgttttgccagtcttatttttagacttagaagtggtttgattgggtccaaggggtctcatgagggaaccagccacacaggcattcaaaagtagacttcccaaaatcaggaagcttcctttccagccaaaagtattaaaaaggtactgattgaaaggagccaatgaacttaagaaaacaggacttcctgccatggccaatccatttgccatgggtcgcttcctatagaagtatttgccaattatggttaaggcgggttgcaggttgaaggctaaacctaaacctgtaatgaatcccatagtgaggtacagctgtaccacgctgctactaaaggaggccaacaccattccaagacagcataataagcctcctgctatcaccaccggccggctgccgtatttattcaccaaaacactacttacaggacctaggcatgatcctgattgagtaaagctgcactgaatcctcaaggatgtgaagatcaaaaagctttcaaatattctacctcctgcgtacataacagccagcataatggatgaaatccatgctatttcactgtaggtagtgtggaatatttgctgaatttctttgaagaatacggtgacagctttggggaatgcataggaaaatccaatggagataaaagctgctccaaccacaatccaaccccatcctccatctggaggtggatgcacaggtggggcacttggcattggtggcatttctgctcctctagtggaaattcaagtaacatacatatctccagagactctgctttgccctcccctctctcttctctcaaatagggcaaagttagttatttctctttttcaagaacctgctttgacgtgcactattagttcatacttttcagagtctaaagtaagcttggcttaaattatatcatgggtcaaagaaggtggccaagtctggcaatttgaactgctaaatttaaccttctcatgtgttgtgttgatgtagccacattttcaagcacattttccattgcgtgatttaatatgcataaaacatattgcaaaaatactgtactatatacattaatagtttagtgactcttcactgagtctgagactaggtaatttgtaagttatgaacaataacaaagaggccagggtcaaagtgttgaatctcttgtgggccagtttaatctatttcttgatcacacataacactccctacatggtcagccactctgtaaatgcatgctctctgtcccaaagagtccccaaccctgtgtgagggtgaatctggtgatagatcattagtaccatcttcgttttagaagaaattactataacctttggaaaaatgcagtggtgtaatttattaaatgcttctcatattctaggtaagcattttgccaaacaatttatacccactaccccattctctaaatgatacatgatagacattatgataaatattttcctatggggacactgaagctcagcgttttgattacttatgtaaggccatatagctgtaaaatatggggtcctggattccaactctagattgtctagattcgaggctcatgttcctctctatcaaacagcatgccagactcctctatcagtggatgagaaatatctgatttcctatgtgaaagatacaattatttagatctaagcactaagcagtagccacttgtaaaatatgcttcccaaagatttgggaaggctgcatttctaaatgtgtataataatgaaataataataaccaggtaataacataaataacctctagaaattttatcta

SEQ ID NO: 11049 - RNA, 6223 nt, Homo sapiens
  source 1..6223: mol_type = other RNA
ctgaatagctgggactacaggtgcacatcaccacatccaggtaattattttactttttgaatcatgatatgtagcaaccaatctgggaattatttattcataaaagataacattttcctgctaactccaacctcagaaaaaatgtattatgcctgactcaaatatgtcattatttttatgagaaaaagagtcatattgaagtaattatgtctatatgtaataattatcattatttgagataatttgcattggggagaaaagcaggcaatcagaaattacatattcaaggctgggcgcagtggctcacgcctgtaatcccagcactttgggaggcagaggcgagtgaatcacctgaggtcagagttcaagaccagcctgaccaacaaggagaaaccccatctctactaaaacaaaacaaaacaaaacaaaacaaaaaaagccacaaaattagccgggcatggtggcacatgcctgtaattccagttactcgggaggctgaggcaggagaattgcttgaacctgggaggcagaggttgtagtaagccgagattgtgccactgcacgccagcctgggcgacaagaacgagactcagtctcaaaaaaaaaaaaaaagaaagaaagaaagaaattacatattcaggttctagcaaatgcagttctctaataaacactaaataaatcataatacaagttacagttaaacctaattgttttactatataggatgtatcttttttgtacctatattttatcttcctttgcttctctggcctctattgggaggcagcacggtagtgaacacctcggggatctttctggttacgtaaacctgagttttaattttggttcatactaccttttaactttgggtagtctgctgagcttgttttttgttttcactcatctgtcatatcaagctagtaataattctgccatggttttggttttcatattgaaaggcattacataagcaaaatgcataacatataaatattagttccctttccactatgcatccaatctccctattaaattaagcctaaaaataataatttttgttttattaaaagccttccacattctacatatgaaagggattttttaaaggtgttttagataaaaaatgtttcaaccaactgaccaagaatatctcttcatatttatgtcatctacataaaaacttacatttatatcatatatcttttagtcttcttttctatattcttgattgtcatgttgtacagccagaaaagaatgagtataaattatctagattttttaaagtgcacattcaaacatagaaaatctaattattttacttgtttcttagtattaggctgaggccaatgagtccatgagctaaagggttgaaacttggcaccaaaaaagtgattgtttatgagtcctgtagatttatactgagaaaacatcatgtcttccaatgtgaaatacactaaaacctgattttttgtctcttaaggtgtgctaggtgaatgcaaaaaggatcaggaaagggggtgaggataggtcaggaaaagtgcaaacacaatgttctattcataaattagtgatggcatatttaaggttaagtagtaaaaaatatggggggctcagttaacacgaatgaaaaaatagttaaagtagccatgaattatctggataccttgatttaatgacaccctttcttctgtacaatttcataatgtgggaatagagattagtggggattgtagtggtataccctgactttgcttcatgatatctcaaatgtttaaaacctattattccctagagaaagaaatatgttcatactaattgttgcagaggcagaagccaaatatatctcctcctccatttatgtgactatatagtaatgaaaatcctaggttgatacacttttctcaatcttggaaagattctgctaaagcagcaaatcttctaacaagttcaagagggtggggagagtgaacaagtagaataatttatattaccctggaacaattctgaatcctgtaggtatttatgtcactgtttcaattgtgttctggtttaactgtcaatatttatgcatagcagttaacgtgtgtgcatatttgtaactgtgcagtgctactgccaggtgtgactgtacaaatcatgtgctttgaatgtgcaagttttactttcttttctaacaatttaatacagtgttagaaataaataacgaatgaagacaaccaaagagcagccagacaaatgtgaactggttttgacgtgacgagaaactcatcagtaagtaaataaacctcctccctggagaaggccactgaaatgcacccaggaggatgtctctactagaaggtaataaaaaatatatataatgtagtctttgacctaaaacctcatgattattactttgccatttatttccccctggtatctgatgttcatattagtttaatgtgccttttcagagaattcaagacactttttggaaagtagaatttttttttgaaaatttatgattggagaggtactacacaatttagaggttacatttcttgacaaatctgagttgaataaaaaagaactaaaaatataaacatagctaattcaagaatcaagatcgggtgaaactaaattaaaaacagccataaagtcccacattttccctaatttatttacctatgatattggcacatcttgttttacttaacatttgaaaaatacaaatatctcttcatatgcaaaagagcaaatgttaaatgaaaaactgaattttatatagcttcctaaatatgagccacatgcttaagcagtgaattaactttatgaatcaaatgtttaatgttaactattacaaaagcctggtatccaggtgcaatctcaccagaaaaaaatagcacctgcctttattacaataaaaaaaatggctaattccctttgacatcttaagagtgacactactttgtcaagcactaaatactttttaaattaatcatgttaaacttcagatttatagatataaatattgtatttataactttagtcataatgtacaatttctttcttgtttaaaagtactttctcactcaaaatggtatttatagtttaaaaagaatatgcctctgtattcaggagtgattcaaattcccagatgttttcacatagttatgaaaatgggaaagtgctgaattaaactgggctgcaatatttcaagttttttgctatcaggttataaactatacctacgattgcaagtcatacagtgcctctatttctagaaggcttttaaagtttcctggcttagttatgtccaaaggcagcaggaagtctcatcagtagagggcagaattttcaagtgctgccattcttatcccaggaggcatttccagtggttgagcacaaggcctgtttgtagtttgcttttgctcttgcattttgtggaagggaaggaactgagagagcttagagggttcattaaaaccacccctcactctcttagtcgtagtcagatggagtattcataacagtaacctccaattaccactatgtgttgggaaaaattagaattcggtctacttacaatcctgccaactaggattttactttgatatttcagtataacagtgaatctggattgatgcctgattaaaataaaatccctgattattactttctggattacgaactaaaatccctgtaaaatcaatggatgtgactcattgttaagagtcatgcagacttttacatattaggtaagaattctaaaaattatttgagggttctattctctagcaccaggtactaatgctccctactcaaaaaaaatcatgtgcatggattaatcaagtctaacagtgctcagatttaatggtttaacattgattttcttttctttgtcaaacttatatatgcaaatatttttatagtagtcagatgttatttttgaataaggatcaccctcatttttacccatgtgcttatctttaaaaccaacattgtaaagtagcacgcagacatatgtttcttttatcttcatggattatttttaccttaaaaataaattatcatttttttttttgaatttgggttttattctccagatactctgtgtacatgtgggtaagtatgtgggagtatgtgtgtttgtgtgtaagaggggataattaattgtctctcaactctatctcatactttaatatcaaataaaaaatgaaatgtataaagggtcactttgtaggattaggcatcctccttctacctacttaaaccaggggtttgggattcagaattctccatataaccaagaccgaaagtcactggaagactttaaaattagtattttaaccaccacacccagagtcaggtatggaaataaacctatagcatggattctttctatgcataatctcaaaatttaactacccaaataagtaagtttttaaaaactaatttaaaatttgccattgaggaaaatatcacctccatccttaattgtgactcctcatttcagctaaaaccttttctaatactttaaaaaaacaaaatgaaaaacaaactcctagataaagtcataaacactgaaatcagagatgtgattcttgttaaatgttagtttctctttctgaggttacactctgtgcatttgaaactttgacgttaacatcttccgaatgtttagatttgctcaagggttcagattctctggtcttctgccttgcattttcctccttcctttcctttgcaagcaatctatagttgatagcattgccaatgagcagccacacgcttgctgctaccacaatagccccacaggacatgtacatgtatttatattctccagttaaatccaccaatttacctgcaagaggagggccaagaagaactgggccacactccacaattgtgacaagtccgacggcactggaaaatcttggtgcacccacgaggtccatgagagtttcaaagagaacactgctaacactcccaaatccaaggccaaaaaatacagcatataataccaggcttgtgtagtcctgtgccagtgggcacaagaggtgacacactccattgaacatgattgcaaaactgaagaagtactgaattcgaggtcgaatatatttggagtttgcaattaatcctacagaaggcctagcaaacatatcaacgaaagccataacagatagcagaaaagctgccgagtactcatcaattccttggtctttagcatatggagccaagaatataatgggggcaaaaaaacctaggaacataatgacatttccagacagatatatcagaaatcctctatgcttaaaaagggagaaatctaaatacttattaactttttcccaagttgatttcttcgttttgattttctttgggcttgaatcatcttctgttttgccagtcttatttttagacttagaagtggtttgattgggtccaaggggtctcatgagggaaccagccacacaggcattcaaaagtagacttcccaaaatcaggaagcttcctttccagccaaaagtattaaaaaggtactgattgaaaggagccaatgaacttaagaaaacaggacttcctgccatggccaatccatttgccatgggtcgcttcctatagaagtatttgccaattatggttaaggcgggttgcaggttgaaggctaaacctaaacctgtaatgaatcccatagtgaggtacagctgtaccacgctgctactaaaggaggccaacaccattccaagacagcataataagcctcctgctatcaccaccggccggctgccgtatttattcaccaaaacactacttacaggacctaggcatgatcctgattgagtaaagctgcactgaatcctcaaggatgtgaagatcaaaaagctttcaaatattctacctcctgcgtacataacagccagcataatggatgaaatccatgctatttcactgtaggtagtgtggaatatttgctgaatttctttgaagaatacggtgacagctttggggaatgcataggaaaatccaatggagataaaagctgctccaaccacaatccaaccccatcctccatctggaggtggatgcacaggtggggcacttggcattggtggcatttctgctcctctagtggaaattcaagtaacctgaatagagagagaacctgcgtttgacacttttctccaggctcagggctaagaagagaggcaactgatcattaacttttagccacaagcaa

SEQ ID NO: 11050 - RNA, 6427 nt, Homo sapiens
  source 1..6427: mol_type = other RNA
ctgaatagctgggactacaggtgcacatcaccacatccaggtaattattttactttttgaatcatgatatgtagcaaccaatctgggaattatttattcataaaagataacattttcctgctaactccaacctcagaaaaaatgtattatgcctgactcaaatatgtcattatttttatgagaaaaagagtcatattgaagtaattatgtctatatgtaataattatcattatttgagataatttgcattggggagaaaagcaggcaatcagaaattacatattcaaggctgggcgcagtggctcacgcctgtaatcccagcactttgggaggcagaggcgagtgaatcacctgaggtcagagttcaagaccagcctgaccaacaaggagaaaccccatctctactaaaacaaaacaaaacaaaacaaaacaaaaaaagccacaaaattagccgggcatggtggcacatgcctgtaattccagttactcgggaggctgaggcaggagaattgcttgaacctgggaggcagaggttgtagtaagccgagattgtgccactgcacgccagcctgggcgacaagaacgagactcagtctcaaaaaaaaaaaaaaagaaagaaagaaagaaattacatattcaggttctagcaaatgcagttctctaataaacactaaataaatcataatacaagttacagttaaacctaattgttttactatataggatgtatcttttttgtacctatattttatcttcctttgcttctctggcctctattgggaggcagcacggtagtgaacacctcggggatctttctggttacgtaaacctgagttttaattttggttcatactaccttttaactttgggtagtctgctgagcttgttttttgttttcactcatctgtcatatcaagctagtaataattctgccatggttttggttttcatattgaaaggcattacataagcaaaatgcataacatataaatattagttccctttccactatgcatccaatctccctattaaattaagcctaaaaataataatttttgttttattaaaagccttccacattctacatatgaaagggattttttaaaggtgttttagataaaaaatgtttcaaccaactgaccaagaatatctcttcatatttatgtcatctacataaaaacttacatttatatcatatatcttttagtcttcttttctatattcttgattgtcatgttgtacagccagaaaagaatgagtataaattatctagattttttaaagtgcacattcaaacatagaaaatctaattattttacttgtttcttagtattaggctgaggccaatgagtccatgagctaaagggttgaaacttggcaccaaaaaagtgattgtttatgagtcctgtagatttatactgagaaaacatcatgtcttccaatgtgaaatacactaaaacctgattttttgtctcttaaggtgtgctaggtgaatgcaaaaaggatcaggaaagggggtgaggataggtcaggaaaagtgcaaacacaatgttctattcataaattagtgatggcatatttaaggttaagtagtaaaaaatatggggggctcagttaacacgaatgaaaaaatagttaaagtagccatgaattatctggataccttgatttaatgacaccctttcttctgtacaatttcataatgtgggaatagagattagtggggattgtagtggtataccctgactttgcttcatgatatctcaaatgtttaaaacctattattccctagagaaagaaatatgttcatactaattgttgcagaggcagaagccaaatatatctcctcctccatttatgtgactatatagtaatgaaaatcctaggttgatacacttttctcaatcttggaaagattctgctaaagcagcaaatcttctaacaagttcaagagggtggggagagtgaacaagtagaataatttatattaccctggaacaattctgaatcctgtaggtatttatgtcactgtttcaattgtgttctggtttaactgtcaatatttatgcatagcagttaacgtgtgtgcatatttgtaactgtgcagtgctactgccaggtgtgactgtacaaatcatgtgctttgaatgtgcaagttttactttcttttctaacaatttaatacagtgttagaaataaataacgaatgaagacaaccaaagagcagccagacaaatgtgaactggttttgacgtgacgagaaactcatcagtaagtaaataaacctcctccctggagaaggccactgaaatgcacccaggaggatgtctctactagaaggtaataaaaaatatatataatgtagtctttgacctaaaacctcatgattattactttgccatttatttccccctggtatctgatgttcatattagtttaatgtgccttttcagagaattcaagacactttttggaaagtagaatttttttttgaaaatttatgattggagaggtactacacaatttagaggttacatttcttgacaaatctgagttgaataaaaaagaactaaaaatataaacatagctaattcaagaatcaagatcgggtgaaactaaattaaaaacagccataaagtcccacattttccctaatttatttacctatgatattggcacatcttgttttacttaacatttgaaaaatacaaatatctcttcatatgcaaaagagcaaatgttaaatgaaaaactgaattttatatagcttcctaaatatgagccacatgcttaagcagtgaattaactttatgaatcaaatgtttaatgttaactattacaaaagcctggtatccaggtgcaatctcaccagaaaaaaatagcacctgcctttattacaataaaaaaaatggctaattccctttgacatcttaagagtgacactactttgtcaagcactaaatactttttaaattaatcatgttaaacttcagatttatagatataaatattgtatttataactttagtcataatgtacaatttctttcttgtttaaaagtactttctcactcaaaatggtatttatagtttaaaaagaatatgcctctgtattcaggagtgattcaaattcccagatgttttcacatagttatgaaaatgggaaagtgctgaattaaactgggctgcaatatttcaagttttttgctatcaggttataaactatacctacgattgcaagtcatacagtgcctctatttctagaaggcttttaaagtttcctggcttagttatgtccaaaggcagcaggaagtctcatcagtagagggcagaattttcaagtgctgccattcttatcccaggaggcatttccagtggttgagcacaaggcctgtttgtagtttgcttttgctcttgcattttgtggaagggaaggaactgagagagcttagagggttcattaaaaccacccctcactctcttagtcgtagtcagatggagtattcataacagtaacctccaattaccactatgtgttgggaaaaattagaattcggtctacttacaatcctgccaactaggattttactttgatatttcagtataacagtgaatctggattgatgcctgattaaaataaaatccctgattattactttctggattacgaactaaaatccctgtaaaatcaatggatgtgactcattgttaagagtcatgcagacttttacatattaggtaagaattctaaaaattatttgagggttctattctctagcaccaggtactaatgctccctactcaaaaaaaatcatgtgcatggattaatcaagtctaacagtgctcagatttaatggtttaacattgattttcttttctttgtcaaacttatatatgcaaatatttttatagtagtcagatgttatttttgaataaggatcaccctcatttttacccatgtgcttatctttaaaaccaacattgtaaagtagcacgcagacatatgtttcttttatcttcatggattatttttaccttaaaaataaattatcatttttttttttgaatttgggttttattctccagatactctgtgtacatgtgggtaagtatgtgggagtatgtgtgtttgtgtgtaagaggggataattaattgtctctcaactctatctcatactttaatatcaaataaaaaatgaaatgtataaagggtcactttgtaggattaggcatcctccttctacctacttaaaccaggggtttgggattcagaattctccatataaccaagaccgaaagtcactggaagactttaaaattagtattttaaccaccacacccagagtcaggtatggaaataaacctatagcatggattctttctatgcataatctcaaaatttaactacccaaataagtaagtttttaaaaactaatttaaaatttgccattgaggaaaatatcacctccatccttaattgtgactcctcatttcagctaaaaccttttctaatactttaaaaaaacaaaatgaaaaacaaactcctagataaagtcataaacactgaaatcagagatgtgattcttgttaaatgttagtttctctttctgaggttacactctgtgcatttgaaactttgacgttaacatcttccgaatgtttagatttgctcaagggttcagattctctggtcttctgccttgcattttcctccttcctttcctttgcaagcaatctatagttgatagcattgccaatgagcagccacacgcttgctgctaccacaatagccccacaggacatgtacatgtatttatattctccagttaaatccaccaatttacctgcaagaggagggccaagaagaactgggccacactccacaattgtgacaagtccgacggcactggaaaatcttggtgcacccacgaggtccatgagagtttcaaagagaacactgctaacactcccaaatccaaggccaaaaaatacagcatataataccaggcttgtgtagtcctgtgccagtgggcacaagaggtgacacactccattgaacatgattgcaaaactgaagaagtactgaattcgaggtcgaatatatttggagtttgcaattaatcctacagaaggcctagcaaacatatcaacgaaagccataacagatagcagaaaagctgccgagtactcatcaattccttggtctttagcatatggagccaagaatataatgggggcaaaaaaacctaggaacataatgacatttccagacagatatatcagaaatcctctatgcttaaaaagggagaaatctaaatacttattaactttttcccaagttgatttcttcgttttgattttctttgggcttgaatcatcttctgttttgccagtcttatttttagacttagaagtggtttgattgggtccaaggggtctcatgagggaaccagccacacaggcattcaaaagtagacttcccaaaatcaggaagcttcctttccagccaaaagtattaaaaaggtactgattgaaaggagccaatgaacttaagaaaacaggacttcctgccatggccaatccatttgccatgggtcgcttcctatagaagtatttgccaattatggttaaggcgggttgcaggttgaaggctaaacctaaacctgtaatgaatcccatagtgaggtacagctgtaccacgctgctactaaaggaggccaacaccattccaagacagcataataagcctcctgctatcaccaccggccggctgccgtatttattcaccaaaacactacttacaggacctaggcatgatcctgattgagtaaagctgcactgaatcctcaaggatgtgaagatcaaaaagctttcaaatattctacctcctgcgtacataacagccagcataatggatgaaatccatgctatttcactgtaggtagtgtggaatatttgctgaatttctttgaagaatacggtgacagctttggggaatgcataggaaaatccaatggagataaaagctgctccaaccacaatccaaccccatcctccatctggaggtggatgcacaggtggggcacttggcattggtggcatttctgctcctctagtggaaattcaagtaacctggcgacaggtgtttagaaacatggtcttccatttcaccaagacataagtttccctgatctatggactcctctccccacctgaggcagaagtttccttgtgaaccattgctctttttagaatcctgaacatacttagttccatctatctctttgtcactcaacactttgtcagctagtctcaggattctatgaccccttcccctagctcacttgagtaatcataatatgggaaaactaatctaaatgccaactctgagaagcggttgcatatattactgtcattcacttgataaa

SEQ ID NO: 11051 - RNA, 6340 nt, Homo sapiens
  source 1..6340: mol_type = other RNA
ctgaatagctgggactacaggtgcacatcaccacatccaggtaattattttactttttgaatcatgatatgtagcaaccaatctgggaattatttattcataaaagataacattttcctgctaactccaacctcagaaaaaatgtattatgcctgactcaaatatgtcattatttttatgagaaaaagagtcatattgaagtaattatgtctatatgtaataattatcattatttgagataatttgcattggggagaaaagcaggcaatcagaaattacatattcaaggctgggcgcagtggctcacgcctgtaatcccagcactttgggaggcagaggcgagtgaatcacctgaggtcagagttcaagaccagcctgaccaacaaggagaaaccccatctctactaaaacaaaacaaaacaaaacaaaacaaaaaaagccacaaaattagccgggcatggtggcacatgcctgtaattccagttactcgggaggctgaggcaggagaattgcttgaacctgggaggcagaggttgtagtaagccgagattgtgccactgcacgccagcctgggcgacaagaacgagactcagtctcaaaaaaaaaaaaaaagaaagaaagaaagaaattacatattcaggttctagcaaatgcagttctctaataaacactaaataaatcataatacaagttacagttaaacctaattgttttactatataggatgtatcttttttgtacctatattttatcttcctttgcttctctggcctctattgggaggcagcacggtagtgaacacctcggggatctttctggttacgtaaacctgagttttaattttggttcatactaccttttaactttgggtagtctgctgagcttgttttttgttttcactcatctgtcatatcaagctagtaataattctgccatggttttggttttcatattgaaaggcattacataagcaaaatgcataacatataaatattagttccctttccactatgcatccaatctccctattaaattaagcctaaaaataataatttttgttttattaaaagccttccacattctacatatgaaagggattttttaaaggtgttttagataaaaaatgtttcaaccaactgaccaagaatatctcttcatatttatgtcatctacataaaaacttacatttatatcatatatcttttagtcttcttttctatattcttgattgtcatgttgtacagccagaaaagaatgagtataaattatctagattttttaaagtgcacattcaaacatagaaaatctaattattttacttgtttcttagtattaggctgaggccaatgagtccatgagctaaagggttgaaacttggcaccaaaaaagtgattgtttatgagtcctgtagatttatactgagaaaacatcatgtcttccaatgtgaaatacactaaaacctgattttttgtctcttaaggtgtgctaggtgaatgcaaaaaggatcaggaaagggggtgaggataggtcaggaaaagtgcaaacacaatgttctattcataaattagtgatggcatatttaaggttaagtagtaaaaaatatggggggctcagttaacacgaatgaaaaaatagttaaagtagccatgaattatctggataccttgatttaatgacaccctttcttctgtacaatttcataatgtgggaatagagattagtggggattgtagtggtataccctgactttgcttcatgatatctcaaatgtttaaaacctattattccctagagaaagaaatatgttcatactaattgttgcagaggcagaagccaaatatatctcctcctccatttatgtgactatatagtaatgaaaatcctaggttgatacacttttctcaatcttggaaagattctgctaaagcagcaaatcttctaacaagttcaagagggtggggagagtgaacaagtagaataatttatattaccctggaacaattctgaatcctgtaggtatttatgtcactgtttcaattgtgttctggtttaactgtcaatatttatgcatagcagttaacgtgtgtgcatatttgtaactgtgcagtgctactgccaggtgtgactgtacaaatcatgtgctttgaatgtgcaagttttactttcttttctaacaatttaatacagtgttagaaataaataacgaatgaagacaaccaaagagcagccagacaaatgtgaactggttttgacgtgacgagaaactcatcagtaagtaaataaacctcctccctggagaaggccactgaaatgcacccaggaggatgtctctactagaaggtaataaaaaatatatataatgtagtctttgacctaaaacctcatgattattactttgccatttatttccccctggtatctgatgttcatattagtttaatgtgccttttcagagaattcaagacactttttggaaagtagaatttttttttgaaaatttatgattggagaggtactacacaatttagaggttacatttcttgacaaatctgagttgaataaaaaagaactaaaaatataaacatagctaattcaagaatcaagatcgggtgaaactaaattaaaaacagccataaagtcccacattttccctaatttatttacctatgatattggcacatcttgttttacttaacatttgaaaaatacaaatatctcttcatatgcaaaagagcaaatgttaaatgaaaaactgaattttatatagcttcctaaatatgagccacatgcttaagcagtgaattaactttatgaatcaaatgtttaatgttaactattacaaaagcctggtatccaggtgcaatctcaccagaaaaaaatagcacctgcctttattacaataaaaaaaatggctaattccctttgacatcttaagagtgacactactttgtcaagcactaaatactttttaaattaatcatgttaaacttcagatttatagatataaatattgtatttataactttagtcataatgtacaatttctttcttgtttaaaagtactttctcactcaaaatggtatttatagtttaaaaagaatatgcctctgtattcaggagtgattcaaattcccagatgttttcacatagttatgaaaatgggaaagtgctgaattaaactgggctgcaatatttcaagttttttgctatcaggttataaactatacctacgattgcaagtcatacagtgcctctatttctagaaggcttttaaagtttcctggcttagttatgtccaaaggcagcaggaagtctcatcagtagagggcagaattttcaagtgctgccattcttatcccaggaggcatttccagtggttgagcacaaggcctgtttgtagtttgcttttgctcttgcattttgtggaagggaaggaactgagagagcttagagggttcattaaaaccacccctcactctcttagtcgtagtcagatggagtattcataacagtaacctccaattaccactatgtgttgggaaaaattagaattcggtctacttacaatcctgccaactaggattttactttgatatttcagtataacagtgaatctggattgatgcctgattaaaataaaatccctgattattactttctggattacgaactaaaatccctgtaaaatcaatggatgtgactcattgttaagagtcatgcagacttttacatattaggtaagaattctaaaaattatttgagggttctattctctagcaccaggtactaatgctccctactcaaaaaaaatcatgtgcatggattaatcaagtctaacagtgctcagatttaatggtttaacattgattttcttttctttgtcaaacttatatatgcaaatatttttatagtagtcagatgttatttttgaataaggatcaccctcatttttacccatgtgcttatctttaaaaccaacattgtaaagtagcacgcagacatatgtttcttttatcttcatggattatttttaccttaaaaataaattatcatttttttttttgaatttgggttttattctccagatactctgtgtacatgtgggtaagtatgtgggagtatgtgtgtttgtgtgtaagaggggataattaattgtctctcaactctatctcatactttaatatcaaataaaaaatgaaatgtataaagggtcactttgtaggattaggcatcctccttctacctacttaaaccaggggtttgggattcagaattctccatataaccaagaccgaaagtcactggaagactttaaaattagtattttaaccaccacacccagagtcaggtatggaaataaacctatagcatggattctttctatgcataatctcaaaatttaactacccaaataagtaagtttttaaaaactaatttaaaatttgccattgaggaaaatatcacctccatccttaattgtgactcctcatttcagctaaaaccttttctaatactttaaaaaaacaaaatgaaaaacaaactcctagataaagtcataaacactgaaatcagagatgtgattcttgttaaatgttagtttctctttctgaggttacactctgtgcatttgaaactttgacgttaacatcttccgaatgtttagatttgctcaagggttcagattctctggtcttctgccttgcattttcctccttcctttcctttgcaagcaatctatagttgatagcattgccaatgagcagccacacgcttgctgctaccacaatagccccacaggacatgtacatgtatttatattctccagttaaatccaccaatttacctgcaagaggagggccaagaagaactgggccacactccacaattgtgacaagtccgacggcactggaaaatcttggtgcacccacgaggtccatgagagtttcaaagagaacactgctaacactcccaaatccaaggccaaaaaatacagcatataataccaggcttgtgtagtcctgtgccagtgggcacaagaggtgacacactccattgaacatgattgcaaaactgaagaagtactgaattcgaggtcgaatatatttggagtttgcaattaatcctacagaaggcctagcaaacatatcaacgaaagccataacagatagcagaaaagctgccgagtactcatcaattccttggtctttagcatatggagccaagaatataatgggggcaaaaaaacctaggaacataatgacatttccagacagatatatcagaaatcctctatgcttaaaaagggagaaatctaaatacttattaactttttcccaagttgatttcttcgttttgattttctttgggcttgaatcatcttctgttttgccagtcttatttttagacttagaagtggtttgattgggtccaaggggtctcatgagggaaccagccacacaggcattcaaaagtagacttcccaaaatcaggaagcttcctttccagccaaaagtattaaaaaggtactgattgaaaggagccaatgaacttaagaaaacaggacttcctgccatggccaatccatttgccatgggtcgcttcctatagaagtatttgccaattatggttaaggcgggttgcaggttgaaggctaaacctaaacctgtaatgaatcccatagtgaggtacagctgtaccacgctgctactaaaggaggccaacaccattccaagacagcataataagcctcctgctatcaccaccggccggctgccgtatttattcaccaaaacactacttacaggacctcctgcgtacataacagccagcataatggatgaaatccatgctatttcactgtaggtagtgtggaatatttgctgaatttctttgaagaatacggtgacagctttggggaatgcataggaaaatccaatggagataaaagctgctccaaccacaatccaaccccatcctccatctggaggtggatgcacaggtggggcacttggcattggtggcatttctgctcctagagtaactctgttggcaccaagagtcccagagtctttggttccccagatcaccttgtttcaggtttcacaggaaagtatcacatcttaagattgactctttatctggtctctggcgcagggtgggcgctgcagccctccgttcccagcaaaccgcagccgattcgcctcgctgtcaacgggtgaatggaattatttatttatttatggcccctgacgtgtcctcgcccgccacagccagcggagaaggaggcggtggcgggaaggggaggcgcggctgctgaacgcccttgtgggtgcggaggagc

SEQ ID NO: 11052 - RNA, 6360 nt, Homo sapiens
  source 1..6360: mol_type = other RNA
ctgaatagctgggactacaggtgcacatcaccacatccaggtaattattttactttttgaatcatgatatgtagcaaccaatctgggaattatttattcataaaagataacattttcctgctaactccaacctcagaaaaaatgtattatgcctgactcaaatatgtcattatttttatgagaaaaagagtcatattgaagtaattatgtctatatgtaataattatcattatttgagataatttgcattggggagaaaagcaggcaatcagaaattacatattcaaggctgggcgcagtggctcacgcctgtaatcccagcactttgggaggcagaggcgagtgaatcacctgaggtcagagttcaagaccagcctgaccaacaaggagaaaccccatctctactaaaacaaaacaaaacaaaacaaaacaaaaaaagccacaaaattagccgggcatggtggcacatgcctgtaattccagttactcgggaggctgaggcaggagaattgcttgaacctgggaggcagaggttgtagtaagccgagattgtgccactgcacgccagcctgggcgacaagaacgagactcagtctcaaaaaaaaaaaaaaagaaagaaagaaagaaattacatattcaggttctagcaaatgcagttctctaataaacactaaataaatcataatacaagttacagttaaacctaattgttttactatataggatgtatcttttttgtacctatattttatcttcctttgcttctctggcctctattgggaggcagcacggtagtgaacacctcggggatctttctggttacgtaaacctgagttttaattttggttcatactaccttttaactttgggtagtctgctgagcttgttttttgttttcactcatctgtcatatcaagctagtaataattctgccatggttttggttttcatattgaaaggcattacataagcaaaatgcataacatataaatattagttccctttccactatgcatccaatctccctattaaattaagcctaaaaataataatttttgttttattaaaagccttccacattctacatatgaaagggattttttaaaggtgttttagataaaaaatgtttcaaccaactgaccaagaatatctcttcatatttatgtcatctacataaaaacttacatttatatcatatatcttttagtcttcttttctatattcttgattgtcatgttgtacagccagaaaagaatgagtataaattatctagattttttaaagtgcacattcaaacatagaaaatctaattattttacttgtttcttagtattaggctgaggccaatgagtccatgagctaaagggttgaaacttggcaccaaaaaagtgattgtttatgagtcctgtagatttatactgagaaaacatcatgtcttccaatgtgaaatacactaaaacctgattttttgtctcttaaggtgtgctaggtgaatgcaaaaaggatcaggaaagggggtgaggataggtcaggaaaagtgcaaacacaatgttctattcataaattagtgatggcatatttaaggttaagtagtaaaaaatatggggggctcagttaacacgaatgaaaaaatagttaaagtagccatgaattatctggataccttgatttaatgacaccctttcttctgtacaatttcataatgtgggaatagagattagtggggattgtagtggtataccctgactttgcttcatgatatctcaaatgtttaaaacctattattccctagagaaagaaatatgttcatactaattgttgcagaggcagaagccaaatatatctcctcctccatttatgtgactatatagtaatgaaaatcctaggttgatacacttttctcaatcttggaaagattctgctaaagcagcaaatcttctaacaagttcaagagggtggggagagtgaacaagtagaataatttatattaccctggaacaattctgaatcctgtaggtatttatgtcactgtttcaattgtgttctggtttaactgtcaatatttatgcatagcagttaacgtgtgtgcatatttgtaactgtgcagtgctactgccaggtgtgactgtacaaatcatgtgctttgaatgtgcaagttttactttcttttctaacaatttaatacagtgttagaaataaataacgaatgaagacaaccaaagagcagccagacaaatgtgaactggttttgacgtgacgagaaactcatcagtaagtaaataaacctcctccctggagaaggccactgaaatgcacccaggaggatgtctctactagaaggtaataaaaaatatatataatgtagtctttgacctaaaacctcatgattattactttgccatttatttccccctggtatctgatgttcatattagtttaatgtgccttttcagagaattcaagacactttttggaaagtagaatttttttttgaaaatttatgattggagaggtactacacaatttagaggttacatttcttgacaaatctgagttgaataaaaaagaactaaaaatataaacatagctaattcaagaatcaagatcgggtgaaactaaattaaaaacagccataaagtcccacattttccctaatttatttacctatgatattggcacatcttgttttacttaacatttgaaaaatacaaatatctcttcatatgcaaaagagcaaatgttaaatgaaaaactgaattttatatagcttcctaaatatgagccacatgcttaagcagtgaattaactttatgaatcaaatgtttaatgttaactattacaaaagcctggtatccaggtgcaatctcaccagaaaaaaatagcacctgcctttattacaataaaaaaaatggctaattccctttgacatcttaagagtgacactactttgtcaagcactaaatactttttaaattaatcatgttaaacttcagatttatagatataaatattgtatttataactttagtcataatgtacaatttctttcttgtttaaaagtactttctcactcaaaatggtatttatagtttaaaaagaatatgcctctgtattcaggagtgattcaaattcccagatgttttcacatagttatgaaaatgggaaagtgctgaattaaactgggctgcaatatttcaagttttttgctatcaggttataaactatacctacgattgcaagtcatacagtgcctctatttctagaaggcttttaaagtttcctggcttagttatgtccaaaggcagcaggaagtctcatcagtagagggcagaattttcaagtgctgccattcttatcccaggaggcatttccagtggttgagcacaaggcctgtttgtagtttgcttttgctcttgcattttgtggaagggaaggaactgagagagcttagagggttcattaaaaccacccctcactctcttagtcgtagtcagatggagtattcataacagtaacctccaattaccactatgtgttgggaaaaattagaattcggtctacttacaatcctgccaactaggattttactttgatatttcagtataacagtgaatctggattgatgcctgattaaaataaaatccctgattattactttctggattacgaactaaaatccctgtaaaatcaatggatgtgactcattgttaagagtcatgcagacttttacatattaggtaagaattctaaaaattatttgagggttctattctctagcaccaggtactaatgctccctactcaaaaaaaatcatgtgcatggattaatcaagtctaacagtgctcagatttaatggtttaacattgattttcttttctttgtcaaacttatatatgcaaatatttttatagtagtcagatgttatttttgaataaggatcaccctcatttttacccatgtgcttatctttaaaaccaacattgtaaagtagcacgcagacatatgtttcttttatcttcatggattatttttaccttaaaaataaattatcatttttttttttgaatttgggttttattctccagatactctgtgtacatgtgggtaagtatgtgggagtatgtgtgtttgtgtgtaagaggggataattaattgtctctcaactctatctcatactttaatatcaaataaaaaatgaaatgtataaagggtcactttgtaggattaggcatcctccttctacctacttaaaccaggggtttgggattcagaattctccatataaccaagaccgaaagtcactggaagactttaaaattagtattttaaccaccacacccagagtcaggtatggaaataaacctatagcatggattctttctatgcataatctcaaaatttaactacccaaataagtaagtttttaaaaactaatttaaaatttgccattgaggaaaatatcacctccatccttaattgtgactcctcatttcagctaaaaccttttctaatactttaaaaaaacaaaatgaaaaacaaactcctagataaagtcataaacactgaaatcagagatgtgattcttgttaaatgttagtttctctttctgaggttacactctgtgcatttgaaactttgacgttaacatcttccgaatgtttagatttgctcaagggttcagattctctggtcttctgccttgcattttcctccttcctttcctttgcaagcaatctatagttgatagcattgccaatgagcagccacacgcttgctgctaccacaatagccccacaggacatgtacatgtatttatattctccagttaaatccaccaatttacctgcaagaggagggccaagaagaactgggccacactccacaattgtgacaagtccgacggcactggaaaatcttggtgcacccacgaggtccatgagagtttcaaagagaacactgctaacactcccaaatccaaggccaaaaaatacagcatataataccaggcttgtgtagtcctgtgccagtgggcacaagaggtgacacactccattgaacatgattgcaaaactgaagaagtactgaattcgaggtcgaatatatttggagtttgcaattaatcctacagaaggcctagcaaacatatcaacgaaagccataacagatagcagaaaagctgccgagtactcatcaattccttggtctttagcatatggagccaagaatataatgggggcaaaaaaacctaggaacataatgacatttccagacagatatatcagaaatcctctatgcttaaaaagggagaaatctaaatacttattaactttttcccaagttgatttcttcgttttgattttctttgggcttgaatcatcttctgttttgccagtcttatttttagacttagaagtggtttgattgggtccaaggggtctcatgagggaaccagccacacaggcattcaaaagtagacttcccaaaatcaggaagcttcctttccagccaaaagtattaaaaaggtactgattgaaaggagccaatgaacttaagaaaacaggacttcctgccatggccaatccatttgccatgggtcgcttcctatagaagtatttgccaattatggttaaggcgggttgcaggttgaaggctaaacctaaacctgtaatgaatcccatagtgaggtacagctgtaccacgctgctactaaaggaggccaacaccattccaagacagcataataagcctcctgctatcaccaccggccggctgccgtatttattcaccaaaacactacttacaggacctcctgcgtacataacagccagcataatggatgaaatccatgctatttcactgtaggtagtgtggaatatttgctgaatttctttgaagaatacggtgacagctttggggaatgcataggaaaatccaatggagataaaagctgctccaaccacaatccaaccccatcctccatctggaggtggatgcacaggtggggcacttggcattggtggcatttctgctcctctagtggaaattcaagtaacagagtaactctgttggcaccaagagtcccagagtctttggttccccagatcaccttgtttcaggtttcacaggaaagtatcacatcttaagattgactctttatctggtctctggcgcagggtgggcgctgcagccctccgttcccagcaaaccgcagccgattcgcctcgctgtcaacgggtgaatggaattatttatttatttatggcccctgacgtgtcctcgcccgccacagccagcggagaaggaggcggtggcgggaaggggaggcgcggctgctgaacgcccttgtgggtgcggaggagc

SEQ ID NO: 11053 - RNA, 7073 nt, Homo sapiens
  source 1..7073: mol_type = other RNA
ctgaatagctgggactacaggtgcacatcaccacatccaggtaattattttactttttgaatcatgatatgtagcaaccaatctgggaattatttattcataaaagataacattttcctgctaactccaacctcagaaaaaatgtattatgcctgactcaaatatgtcattatttttatgagaaaaagagtcatattgaagtaattatgtctatatgtaataattatcattatttgagataatttgcattggggagaaaagcaggcaatcagaaattacatattcaaggctgggcgcagtggctcacgcctgtaatcccagcactttgggaggcagaggcgagtgaatcacctgaggtcagagttcaagaccagcctgaccaacaaggagaaaccccatctctactaaaacaaaacaaaacaaaacaaaacaaaaaaagccacaaaattagccgggcatggtggcacatgcctgtaattccagttactcgggaggctgaggcaggagaattgcttgaacctgggaggcagaggttgtagtaagccgagattgtgccactgcacgccagcctgggcgacaagaacgagactcagtctcaaaaaaaaaaaaaaagaaagaaagaaagaaattacatattcaggttctagcaaatgcagttctctaataaacactaaataaatcataatacaagttacagttaaacctaattgttttactatataggatgtatcttttttgtacctatattttatcttcctttgcttctctggcctctattgggaggcagcacggtagtgaacacctcggggatctttctggttacgtaaacctgagttttaattttggttcatactaccttttaactttgggtagtctgctgagcttgttttttgttttcactcatctgtcatatcaagctagtaataattctgccatggttttggttttcatattgaaaggcattacataagcaaaatgcataacatataaatattagttccctttccactatgcatccaatctccctattaaattaagcctaaaaataataatttttgttttattaaaagccttccacattctacatatgaaagggattttttaaaggtgttttagataaaaaatgtttcaaccaactgaccaagaatatctcttcatatttatgtcatctacataaaaacttacatttatatcatatatcttttagtcttcttttctatattcttgattgtcatgttgtacagccagaaaagaatgagtataaattatctagattttttaaagtgcacattcaaacatagaaaatctaattattttacttgtttcttagtattaggctgaggccaatgagtccatgagctaaagggttgaaacttggcaccaaaaaagtgattgtttatgagtcctgtagatttatactgagaaaacatcatgtcttccaatgtgaaatacactaaaacctgattttttgtctcttaaggtgtgctaggtgaatgcaaaaaggatcaggaaagggggtgaggataggtcaggaaaagtgcaaacacaatgttctattcataaattagtgatggcatatttaaggttaagtagtaaaaaatatggggggctcagttaacacgaatgaaaaaatagttaaagtagccatgaattatctggataccttgatttaatgacaccctttcttctgtacaatttcataatgtgggaatagagattagtggggattgtagtggtataccctgactttgcttcatgatatctcaaatgtttaaaacctattattccctagagaaagaaatatgttcatactaattgttgcagaggcagaagccaaatatatctcctcctccatttatgtgactatatagtaatgaaaatcctaggttgatacacttttctcaatcttggaaagattctgctaaagcagcaaatcttctaacaagttcaagagggtggggagagtgaacaagtagaataatttatattaccctggaacaattctgaatcctgtaggtatttatgtcactgtttcaattgtgttctggtttaactgtcaatatttatgcatagcagttaacgtgtgtgcatatttgtaactgtgcagtgctactgccaggtgtgactgtacaaatcatgtgctttgaatgtgcaagttttactttcttttctaacaatttaatacagtgttagaaataaataacgaatgaagacaaccaaagagcagccagacaaatgtgaactggttttgacgtgacgagaaactcatcagtaagtaaataaacctcctccctggagaaggccactgaaatgcacccaggaggatgtctctactagaaggtaataaaaaatatatataatgtagtctttgacctaaaacctcatgattattactttgccatttatttccccctggtatctgatgttcatattagtttaatgtgccttttcagagaattcaagacactttttggaaagtagaatttttttttgaaaatttatgattggagaggtactacacaatttagaggttacatttcttgacaaatctgagttgaataaaaaagaactaaaaatataaacatagctaattcaagaatcaagatcgggtgaaactaaattaaaaacagccataaagtcccacattttccctaatttatttacctatgatattggcacatcttgttttacttaacatttgaaaaatacaaatatctcttcatatgcaaaagagcaaatgttaaatgaaaaactgaattttatatagcttcctaaatatgagccacatgcttaagcagtgaattaactttatgaatcaaatgtttaatgttaactattacaaaagcctggtatccaggtgcaatctcaccagaaaaaaatagcacctgcctttattacaataaaaaaaatggctaattccctttgacatcttaagagtgacactactttgtcaagcactaaatactttttaaattaatcatgttaaacttcagatttatagatataaatattgtatttataactttagtcataatgtacaatttctttcttgtttaaaagtactttctcactcaaaatggtatttatagtttaaaaagaatatgcctctgtattcaggagtgattcaaattcccagatgttttcacatagttatgaaaatgggaaagtgctgaattaaactgggctgcaatatttcaagttttttgctatcaggttataaactatacctacgattgcaagtcatacagtgcctctatttctagaaggcttttaaagtttcctggcttagttatgtccaaaggcagcaggaagtctcatcagtagagggcagaattttcaagtgctgccattcttatcccaggaggcatttccagtggttgagcacaaggcctgtttgtagtttgcttttgctcttgcattttgtggaagggaaggaactgagagagcttagagggttcattaaaaccacccctcactctcttagtcgtagtcagatggagtattcataacagtaacctccaattaccactatgtgttgggaaaaattagaattcggtctacttacaatcctgccaactaggattttactttgatatttcagtataacagtgaatctggattgatgcctgattaaaataaaatccctgattattactttctggattacgaactaaaatccctgtaaaatcaatggatgtgactcattgttaagagtcatgcagacttttacatattaggtaagaattctaaaaattatttgagggttctattctctagcaccaggtactaatgctccctactcaaaaaaaatcatgtgcatggattaatcaagtctaacagtgctcagatttaatggtttaacattgattttcttttctttgtcaaacttatatatgcaaatatttttatagtagtcagatgttatttttgaataaggatcaccctcatttttacccatgtgcttatctttaaaaccaacattgtaaagtagcacgcagacatatgtttcttttatcttcatggattatttttaccttaaaaataaattatcatttttttttttgaatttgggttttattctccagatactctgtgtacatgtgggtaagtatgtgggagtatgtgtgtttgtgtgtaagaggggataattaattgtctctcaactctatctcatactttaatatcaaataaaaaatgaaatgtataaagggtcactttgtaggattaggcatcctccttctacctacttaaaccaggggtttgggattcagaattctccatataaccaagaccgaaagtcactggaagactttaaaattagtattttaaccaccacacccagagtcaggtatggaaataaacctatagcatggattctttctatgcataatctcaaaatttaactacccaaataagtaagtttttaaaaactaatttaaaatttgccattgaggaaaatatcacctccatccttaattgtgactcctcatttcagctaaaaccttttctaatactttaaaaaaacaaaatgaaaaacaaactcctagataaagtcataaacactgaaatcagagatgtgattcttgttaaatgttagtttctctttctgaggttacactctgtgcatttgaaactttgacgttaacatcttccgaatgtttagatttgctcaagggttcagattctctggtcttctgccttgcattttcctccttcctttcctttgcaagcaatctatagttgatagcattgccaatgagcagccacacgcttgctgctaccacaatagccccacaggacatgtacatgtatttatattctccagttaaatccaccaatttacctgcaagaggagggccaagaagaactgggccacactccacaattgtgacaagtccgacggcactggaaaatcttggtgcacccacgaggtccatgagagtttcaaagagaacactgctaacactcccaaatccaaggccaaaaaatacagcatataataccaggcttgtgtagtcctgtgccagtgggcacaagaggtgacacactccattgaacatgattgcaaaactgaagaagtactgaattcgaggtcgaatatatttggagtttgcaattaatcctacagaaggcctagcaaacatatcaacgaaagccataacagatagcagaaaagctgccgagtactcatcaattccttggtctttagcatatggagccaagaatataatgggggcaaaaaaacctaggaacataatgacatttccagacagatatatcagaaatcctctatgcttaaaaagggagaaatctaaatacttattaactttttcccaagttgatttcttcgttttgattttctttgggcttgaatcatcttctgttttgccagtcttatttttagacttagaagtggtttgattgggtccaaggggtctcatgagggaaccagccacacaggcattcaaaagtagacttcccaaaatcaggaagcttcctttccagccaaaagtattaaaaaggtactgattgaaaggagccaatgaacttaagaaaacaggacttcctgccatggccaatccatttgccatgggtcgcttcctatagaagtatttgccaattatggttaaggcgggttgcaggttgaaggctaaacctaaacctgtaatgaatcccatagtgaggtacagctgtaccacgctgctactaaaggaggccaacaccattccaagacagcataataagcctcctgctatcaccaccggccggctgccgtatttattcaccaaaacactacttacaggacctcctgcgtacataacagccagcataatggatgaaatccatgctatttcactgtaggtagtgtggaatatttgctgaatttctttgaagaatacggtgacagctttggggaatgcataggaaaatccaatggagataaaagctgctccaaccacaatccaaccccatcctccatctggaggtggatgcacaggtggggcacttggcattggtggcatttctgctcctctagtggaaattcaagtaacatacatatctccagagactctgctttgccctcccctctctcttctctcaaatagggcaaagttagttatttctctttttcaagaacctgctttgacgtgcactattagttcatacttttcagagtctaaagtaagcttggcttaaattatatcatgggtcaaagaaggtggccaagtctggcaatttgaactgctaaatttaaccttctcatgtgttgtgttgatgtagccacattttcaagcacattttccattgcgtgatttaatatgcataaaacatattgcaaaaatactgtactatatacattaatagtttagtgactcttcactgagtctgagactaggtaatttgtaagttatgaacaataacaaagaggccagggtcaaagtgttgaatctcttgtgggccagtttaatctatttcttgatcacacataacactccctacatggtcagccactctgtaaatgcatgctctctgtcccaaagagtccccaaccctgtgtgagggtgaatctggtgatagatcattagtaccatcttcgttttagaagaaattactataacctttggaaaaatgcagtggtgtaatttattaaatgcttctcatattctaggtaagcattttgccaaacaatttatacccactaccccattctctaaatgatacatgatagacattatgataaatattttcctatggggacactgaagctcagcgttttgattacttatgtaaggccatatagctgtaaaatatggggtcctggattccaactctagattgtctagattcgaggctcatgttcctctctatcaaacagcatgccagactcctctatcagtggatgagaaatatctgatttcctatgtgaaagatacaattatttagatctaagcactaagcagtagccacttgtaaaatatgcttcccaaagatttgggaaggctgcatttctaaatgtgtataataatgaaataataataaccaggtaataacataaataacctctagaaatt

SEQ ID NO: 11054 - RNA, 6123 nt, Homo sapiens
  source 1..6123: mol_type = other RNA
ctgaatagctgggactacaggtgcacatcaccacatccaggtaattattttactttttgaatcatgatatgtagcaaccaatctgggaattatttattcataaaagataacattttcctgctaactccaacctcagaaaaaatgtattatgcctgactcaaatatgtcattatttttatgagaaaaagagtcatattgaagtaattatgtctatatgtaataattatcattatttgagataatttgcattggggagaaaagcaggcaatcagaaattacatattcaaggctgggcgcagtggctcacgcctgtaatcccagcactttgggaggcagaggcgagtgaatcacctgaggtcagagttcaagaccagcctgaccaacaaggagaaaccccatctctactaaaacaaaacaaaacaaaacaaaacaaaaaaagccacaaaattagccgggcatggtggcacatgcctgtaattccagttactcgggaggctgaggcaggagaattgcttgaacctgggaggcagaggttgtagtaagccgagattgtgccactgcacgccagcctgggcgacaagaacgagactcagtctcaaaaaaaaaaaaaaagaaagaaagaaagaaattacatattcaggttctagcaaatgcagttctctaataaacactaaataaatcataatacaagttacagttaaacctaattgttttactatataggatgtatcttttttgtacctatattttatcttcctttgcttctctggcctctattgggaggcagcacggtagtgaacacctcggggatctttctggttacgtaaacctgagttttaattttggttcatactaccttttaactttgggtagtctgctgagcttgttttttgttttcactcatctgtcatatcaagctagtaataattctgccatggttttggttttcatattgaaaggcattacataagcaaaatgcataacatataaatattagttccctttccactatgcatccaatctccctattaaattaagcctaaaaataataatttttgttttattaaaagccttccacattctacatatgaaagggattttttaaaggtgttttagataaaaaatgtttcaaccaactgaccaagaatatctcttcatatttatgtcatctacataaaaacttacatttatatcatatatcttttagtcttcttttctatattcttgattgtcatgttgtacagccagaaaagaatgagtataaattatctagattttttaaagtgcacattcaaacatagaaaatctaattattttacttgtttcttagtattaggctgaggccaatgagtccatgagctaaagggttgaaacttggcaccaaaaaagtgattgtttatgagtcctgtagatttatactgagaaaacatcatgtcttccaatgtgaaatacactaaaacctgattttttgtctcttaaggtgtgctaggtgaatgcaaaaaggatcaggaaagggggtgaggataggtcaggaaaagtgcaaacacaatgttctattcataaattagtgatggcatatttaaggttaagtagtaaaaaatatggggggctcagttaacacgaatgaaaaaatagttaaagtagccatgaattatctggataccttgatttaatgacaccctttcttctgtacaatttcataatgtgggaatagagattagtggggattgtagtggtataccctgactttgcttcatgatatctcaaatgtttaaaacctattattccctagagaaagaaatatgttcatactaattgttgcagaggcagaagccaaatatatctcctcctccatttatgtgactatatagtaatgaaaatcctaggttgatacacttttctcaatcttggaaagattctgctaaagcagcaaatcttctaacaagttcaagagggtggggagagtgaacaagtagaataatttatattaccctggaacaattctgaatcctgtaggtatttatgtcactgtttcaattgtgttctggtttaactgtcaatatttatgcatagcagttaacgtgtgtgcatatttgtaactgtgcagtgctactgccaggtgtgactgtacaaatcatgtgctttgaatgtgcaagttttactttcttttctaacaatttaatacagtgttagaaataaataacgaatgaagacaaccaaagagcagccagacaaatgtgaactggttttgacgtgacgagaaactcatcagtaagtaaataaacctcctccctggagaaggccactgaaatgcacccaggaggatgtctctactagaaggtaataaaaaatatatataatgtagtctttgacctaaaacctcatgattattactttgccatttatttccccctggtatctgatgttcatattagtttaatgtgccttttcagagaattcaagacactttttggaaagtagaatttttttttgaaaatttatgattggagaggtactacacaatttagaggttacatttcttgacaaatctgagttgaataaaaaagaactaaaaatataaacatagctaattcaagaatcaagatcgggtgaaactaaattaaaaacagccataaagtcccacattttccctaatttatttacctatgatattggcacatcttgttttacttaacatttgaaaaatacaaatatctcttcatatgcaaaagagcaaatgttaaatgaaaaactgaattttatatagcttcctaaatatgagccacatgcttaagcagtgaattaactttatgaatcaaatgtttaatgttaactattacaaaagcctggtatccaggtgcaatctcaccagaaaaaaatagcacctgcctttattacaataaaaaaaatggctaattccctttgacatcttaagagtgacactactttgtcaagcactaaatactttttaaattaatcatgttaaacttcagatttatagatataaatattgtatttataactttagtcataatgtacaatttctttcttgtttaaaagtactttctcactcaaaatggtatttatagtttaaaaagaatatgcctctgtattcaggagtgattcaaattcccagatgttttcacatagttatgaaaatgggaaagtgctgaattaaactgggctgcaatatttcaagttttttgctatcaggttataaactatacctacgattgcaagtcatacagtgcctctatttctagaaggcttttaaagtttcctggcttagttatgtccaaaggcagcaggaagtctcatcagtagagggcagaattttcaagtgctgccattcttatcccaggaggcatttccagtggttgagcacaaggcctgtttgtagtttgcttttgctcttgcattttgtggaagggaaggaactgagagagcttagagggttcattaaaaccacccctcactctcttagtcgtagtcagatggagtattcataacagtaacctccaattaccactatgtgttgggaaaaattagaattcggtctacttacaatcctgccaactaggattttactttgatatttcagtataacagtgaatctggattgatgcctgattaaaataaaatccctgattattactttctggattacgaactaaaatccctgtaaaatcaatggatgtgactcattgttaagagtcatgcagacttttacatattaggtaagaattctaaaaattatttgagggttctattctctagcaccaggtactaatgctccctactcaaaaaaaatcatgtgcatggattaatcaagtctaacagtgctcagatttaatggtttaacattgattttcttttctttgtcaaacttatatatgcaaatatttttatagtagtcagatgttatttttgaataaggatcaccctcatttttacccatgtgcttatctttaaaaccaacattgtaaagtagcacgcagacatatgtttcttttatcttcatggattatttttaccttaaaaataaattatcatttttttttttgaatttgggttttattctccagatactctgtgtacatgtgggtaagtatgtgggagtatgtgtgtttgtgtgtaagaggggataattaattgtctctcaactctatctcatactttaatatcaaataaaaaatgaaatgtataaagggtcactttgtaggattaggcatcctccttctacctacttaaaccaggggtttgggattcagaattctccatataaccaagaccgaaagtcactggaagactttaaaattagtattttaaccaccacacccagagtcaggtatggaaataaacctatagcatggattctttctatgcataatctcaaaatttaactacccaaataagtaagtttttaaaaactaatttaaaatttgccattgaggaaaatatcacctccatccttaattgtgactcctcatttcagctaaaaccttttctaatactttaaaaaaacaaaatgaaaaacaaactcctagataaagtcataaacactgaaatcagagatgtgattcttgttaaatgttagtttctctttctgaggttacactctgtgcatttgaaactttgacgttaacatcttccgaatgtttagatttgctcaagggttcagattctctggtcttctgccttgcattttcctccttcctttcctttgcaagcaatctatagttgatagcattgccaatgagcagccacacgcttgctgctaccacaatagccccacaggacatgtacatgtatttatattctccagttaaatccaccaatttacctgcaagaggagggccaagaagaactgggccacactccacaattgtgacaagtccgacggcactggaaaatcttggtgcacccacgaggtccatgagagtttcaaagagaacactgctaacactcccaaatccaaggccaaaaaatacagcatataataccaggcttgtgtagtcctgtgccagtgggcacaagaggtgacacactccattgaacatgattgcaaaactgaagaagtactgaattcgaggtcgaatatatttggagtttgcaattaatcctacagaaggcctagcaaacatatcaacgaaagccataacagatagcagaaaagctgccgagtactcatcaattccttggtctttagcatatggagccaagaatataatgggggcaaaaaaacctaggaacataatgacatttccagacagatatatcagaaatcctctatgcttaaaaagggagaaatctaaatacttattaactttttcccaagttgatttcttcgttttgattttctttgggcttgaatcatcttctgttttgccagtcttatttttagacttagaagtggtttgattgggtccaaggggtctcatgagggaaccagccacacaggcattcaaaagtagacttcccaaaatcaggaagcttcctttccagccaaaagtattaaaaaggtactgattgaaaggagccaatgaacttaagaaaacaggacttcctgccatggccaatccatttgccatgggtcgcttcctatagaagtatttgccaattatggttaaggcgggttgcaggttgaaggctaaacctaaacctgtaatgaatcccatagtgaggtacagctgtaccacgctgctactaaaggaggccaacaccattccaagacagcataataagcctcctgctatcaccaccggccggctgccgtatttattcaccaaaacactacttacaggacctcctgcgtacataacagccagcataatggatgaaatccatgctatttcactgtaggtagtgtggaatatttgctgaatttctttgaagaatacggtgacagctttggggaatgcataggaaaatccaatggagataaaagctgctccaaccacaatccaaccccatcctccatctggaggtggatgcacaggtggggcacttggcattggtggcatttctgctcctctagtggaaattcaagtaacctgaatagagagagaacctgcgtttgacacttttctccaggctcagggctaagaagagaggcaactgatc

SEQ ID NO: 11055 - RNA, 6154 nt, Homo sapiens
  source 1..6154: mol_type = other RNA
ctgaatagctgggactacaggtgcacatcaccacatccaggtaattattttactttttgaatcatgatatgtagcaaccaatctgggaattatttattcataaaagataacattttcctgctaactccaacctcagaaaaaatgtattatgcctgactcaaatatgtcattatttttatgagaaaaagagtcatattgaagtaattatgtctatatgtaataattatcattatttgagataatttgcattggggagaaaagcaggcaatcagaaattacatattcaaggctgggcgcagtggctcacgcctgtaatcccagcactttgggaggcagaggcgagtgaatcacctgaggtcagagttcaagaccagcctgaccaacaaggagaaaccccatctctactaaaacaaaacaaaacaaaacaaaacaaaaaaagccacaaaattagccgggcatggtggcacatgcctgtaattccagttactcgggaggctgaggcaggagaattgcttgaacctgggaggcagaggttgtagtaagccgagattgtgccactgcacgccagcctgggcgacaagaacgagactcagtctcaaaaaaaaaaaaaaagaaagaaagaaagaaattacatattcaggttctagcaaatgcagttctctaataaacactaaataaatcataatacaagttacagttaaacctaattgttttactatataggatgtatcttttttgtacctatattttatcttcctttgcttctctggcctctattgggaggcagcacggtagtgaacacctcggggatctttctggttacgtaaacctgagttttaattttggttcatactaccttttaactttgggtagtctgctgagcttgttttttgttttcactcatctgtcatatcaagctagtaataattctgccatggttttggttttcatattgaaaggcattacataagcaaaatgcataacatataaatattagttccctttccactatgcatccaatctccctattaaattaagcctaaaaataataatttttgttttattaaaagccttccacattctacatatgaaagggattttttaaaggtgttttagataaaaaatgtttcaaccaactgaccaagaatatctcttcatatttatgtcatctacataaaaacttacatttatatcatatatcttttagtcttcttttctatattcttgattgtcatgttgtacagccagaaaagaatgagtataaattatctagattttttaaagtgcacattcaaacatagaaaatctaattattttacttgtttcttagtattaggctgaggccaatgagtccatgagctaaagggttgaaacttggcaccaaaaaagtgattgtttatgagtcctgtagatttatactgagaaaacatcatgtcttccaatgtgaaatacactaaaacctgattttttgtctcttaaggtgtgctaggtgaatgcaaaaaggatcaggaaagggggtgaggataggtcaggaaaagtgcaaacacaatgttctattcataaattagtgatggcatatttaaggttaagtagtaaaaaatatggggggctcagttaacacgaatgaaaaaatagttaaagtagccatgaattatctggataccttgatttaatgacaccctttcttctgtacaatttcataatgtgggaatagagattagtggggattgtagtggtataccctgactttgcttcatgatatctcaaatgtttaaaacctattattccctagagaaagaaatatgttcatactaattgttgcagaggcagaagccaaatatatctcctcctccatttatgtgactatatagtaatgaaaatcctaggttgatacacttttctcaatcttggaaagattctgctaaagcagcaaatcttctaacaagttcaagagggtggggagagtgaacaagtagaataatttatattaccctggaacaattctgaatcctgtaggtatttatgtcactgtttcaattgtgttctggtttaactgtcaatatttatgcatagcagttaacgtgtgtgcatatttgtaactgtgcagtgctactgccaggtgtgactgtacaaatcatgtgctttgaatgtgcaagttttactttcttttctaacaatttaatacagtgttagaaataaataacgaatgaagacaaccaaagagcagccagacaaatgtgaactggttttgacgtgacgagaaactcatcagtaagtaaataaacctcctccctggagaaggccactgaaatgcacccaggaggatgtctctactagaaggtaataaaaaatatatataatgtagtctttgacctaaaacctcatgattattactttgccatttatttccccctggtatctgatgttcatattagtttaatgtgccttttcagagaattcaagacactttttggaaagtagaatttttttttgaaaatttatgattggagaggtactacacaatttagaggttacatttcttgacaaatctgagttgaataaaaaagaactaaaaatataaacatagctaattcaagaatcaagatcgggtgaaactaaattaaaaacagccataaagtcccacattttccctaatttatttacctatgatattggcacatcttgttttacttaacatttgaaaaatacaaatatctcttcatatgcaaaagagcaaatgttaaatgaaaaactgaattttatatagcttcctaaatatgagccacatgcttaagcagtgaattaactttatgaatcaaatgtttaatgttaactattacaaaagcctggtatccaggtgcaatctcaccagaaaaaaatagcacctgcctttattacaataaaaaaaatggctaattccctttgacatcttaagagtgacactactttgtcaagcactaaatactttttaaattaatcatgttaaacttcagatttatagatataaatattgtatttataactttagtcataatgtacaatttctttcttgtttaaaagtactttctcactcaaaatggtatttatagtttaaaaagaatatgcctctgtattcaggagtgattcaaattcccagatgttttcacatagttatgaaaatgggaaagtgctgaattaaactgggctgcaatatttcaagttttttgctatcaggttataaactatacctacgattgcaagtcatacagtgcctctatttctagaaggcttttaaagtttcctggcttagttatgtccaaaggcagcaggaagtctcatcagtagagggcagaattttcaagtgctgccattcttatcccaggaggcatttccagtggttgagcacaaggcctgtttgtagtttgcttttgctcttgcattttgtggaagggaaggaactgagagagcttagagggttcattaaaaccacccctcactctcttagtcgtagtcagatggagtattcataacagtaacctccaattaccactatgtgttgggaaaaattagaattcggtctacttacaatcctgccaactaggattttactttgatatttcagtataacagtgaatctggattgatgcctgattaaaataaaatccctgattattactttctggattacgaactaaaatccctgtaaaatcaatggatgtgactcattgttaagagtcatgcagacttttacatattaggtaagaattctaaaaattatttgagggttctattctctagcaccaggtactaatgctccctactcaaaaaaaatcatgtgcatggattaatcaagtctaacagtgctcagatttaatggtttaacattgattttcttttctttgtcaaacttatatatgcaaatatttttatagtagtcagatgttatttttgaataaggatcaccctcatttttacccatgtgcttatctttaaaaccaacattgtaaagtagcacgcagacatatgtttcttttatcttcatggattatttttaccttaaaaataaattatcatttttttttttgaatttgggttttattctccagatactctgtgtacatgtgggtaagtatgtgggagtatgtgtgtttgtgtgtaagaggggataattaattgtctctcaactctatctcatactttaatatcaaataaaaaatgaaatgtataaagggtcactttgtaggattaggcatcctccttctacctacttaaaccaggggtttgggattcagaattctccatataaccaagaccgaaagtcactggaagactttaaaattagtattttaaccaccacacccagagtcaggtatggaaataaacctatagcatggattctttctatgcataatctcaaaatttaactacccaaataagtaagtttttaaaaactaatttaaaatttgccattgaggaaaatatcacctccatccttaattgtgactcctcatttcagctaaaaccttttctaatactttaaaaaaacaaaatgaaaaacaaactcctagataaagtcataaacactgaaatcagagatgtgattcttgttaaatgttagtttctctttctgaggttacactctgtgcatttgaaactttgacgttaacatcttccgaatgtttagatttgctcaagggttcagattctctggtcttctgccttgcattttcctccttcctttcctttgcaagcaatctatagttgatagcattgccaatgagcagccacacgcttgctgctaccacaatagccccacaggacatgtacatgtatttatattctccagttaaatccaccaatttacctgcaagaggagggccaagaagaactgggccacactccacaattgtgacaagtccgacggcactggaaaatcttggtgcacccacgaggtccatgagagtttcaaagagaacactgctaacactcccaaatccaaggccaaaaaatacagcatataataccaggcttgtgtagtcctgtgccagtgggcacaagaggtgacacactccattgaacatgattgcaaaactgaagaagtactgaattcgaggtcgaatatatttggagtttgcaattaatcctacagaaggcctagcaaacatatcaacgaaagccataacagatagcagaaaagctgccgagtactcatcaattccttggtctttagcatatggagccaagaatataatgggggcaaaaaaacctaggaacataatgacatttccagacagatatatcagaaatcctctatgcttaaaaagggagaaatctaaatacttattaactttttcccaagttgatttcttcgttttgattttctttgggcttgaatcatcttctgttttgccagtcttatttttagacttagaagtggtttgattgggtccaaggggtctcatgagggaaccagccacacaggcattcaaaagtagacttcccaaaatcaggaagcttcctttccagccaaaagtattaaaaaggtactgattgaaaggagccaatgaacttaagaaaacaggacttcctgccatggccaatccatttgccatgggtcgcttcctatagaagtatttgccaattatggttaaggcgggttgcaggttgaaggctaaacctaaacctgtaatgaatcccatagtgaggtacagctgtaccacgctgctactaaaggaggccaacaccattccaagacagcataataagcctcctgctatcaccaccggccggctgccgtatttattcaccaaaacactacttacaggacctcctgcgtacataacagccagcataatggatgaaatccatgctatttcactgtaggtagtgtggaatatttgctgaatttctttgaagaatacggtgacagctttggggaatgcataggaaaatccaatggagataaaagctgctccaaccacaatccaaccccatcctccatctggaggtggatgcacaggtggggcacttggcattggtggcatttctgctcctctagtggaaattcaagtaacctggcgacaggtgtttagaaacatggtcttccatttcaccaagacataagtttccctgatctatggactcctctccccacctgaggcagaagtttccttgt

SEQ ID NO: 11056 - RNA, 6430 nt, Homo sapiens
  source 1..6430: mol_type = other RNA
ctgaatagctgggactacaggtgcacatcaccacatccaggtaattattttactttttgaatcatgatatgtagcaaccaatctgggaattatttattcataaaagataacattttcctgctaactccaacctcagaaaaaatgtattatgcctgactcaaatatgtcattatttttatgagaaaaagagtcatattgaagtaattatgtctatatgtaataattatcattatttgagataatttgcattggggagaaaagcaggcaatcagaaattacatattcaaggctgggcgcagtggctcacgcctgtaatcccagcactttgggaggcagaggcgagtgaatcacctgaggtcagagttcaagaccagcctgaccaacaaggagaaaccccatctctactaaaacaaaacaaaacaaaacaaaacaaaaaaagccacaaaattagccgggcatggtggcacatgcctgtaattccagttactcgggaggctgaggcaggagaattgcttgaacctgggaggcagaggttgtagtaagccgagattgtgccactgcacgccagcctgggcgacaagaacgagactcagtctcaaaaaaaaaaaaaaagaaagaaagaaagaaattacatattcaggttctagcaaatgcagttctctaataaacactaaataaatcataatacaagttacagttaaacctaattgttttactatataggatgtatcttttttgtacctatattttatcttcctttgcttctctggcctctattgggaggcagcacggtagtgaacacctcggggatctttctggttacgtaaacctgagttttaattttggttcatactaccttttaactttgggtagtctgctgagcttgttttttgttttcactcatctgtcatatcaagctagtaataattctgccatggttttggttttcatattgaaaggcattacataagcaaaatgcataacatataaatattagttccctttccactatgcatccaatctccctattaaattaagcctaaaaataataatttttgttttattaaaagccttccacattctacatatgaaagggattttttaaaggtgttttagataaaaaatgtttcaaccaactgaccaagaatatctcttcatatttatgtcatctacataaaaacttacatttatatcatatatcttttagtcttcttttctatattcttgattgtcatgttgtacagccagaaaagaatgagtataaattatctagattttttaaagtgcacattcaaacatagaaaatctaattattttacttgtttcttagtattaggctgaggccaatgagtccatgagctaaagggttgaaacttggcaccaaaaaagtgattgtttatgagtcctgtagatttatactgagaaaacatcatgtcttccaatgtgaaatacactaaaacctgattttttgtctcttaaggtgtgctaggtgaatgcaaaaaggatcaggaaagggggtgaggataggtcaggaaaagtgcaaacacaatgttctattcataaattagtgatggcatatttaaggttaagtagtaaaaaatatggggggctcagttaacacgaatgaaaaaatagttaaagtagccatgaattatctggataccttgatttaatgacaccctttcttctgtacaatttcataatgtgggaatagagattagtggggattgtagtggtataccctgactttgcttcatgatatctcaaatgtttaaaacctattattccctagagaaagaaatatgttcatactaattgttgcagaggcagaagccaaatatatctcctcctccatttatgtgactatatagtaatgaaaatcctaggttgatacacttttctcaatcttggaaagattctgctaaagcagcaaatcttctaacaagttcaagagggtggggagagtgaacaagtagaataatttatattaccctggaacaattctgaatcctgtaggtatttatgtcactgtttcaattgtgttctggtttaactgtcaatatttatgcatagcagttaacgtgtgtgcatatttgtaactgtgcagtgctactgccaggtgtgactgtacaaatcatgtgctttgaatgtgcaagttttactttcttttctaacaatttaatacagtgttagaaataaataacgaatgaagacaaccaaagagcagccagacaaatgtgaactggttttgacgtgacgagaaactcatcagtaagtaaataaacctcctccctggagaaggccactgaaatgcacccaggaggatgtctctactagaaggtaataaaaaatatatataatgtagtctttgacctaaaacctcatgattattactttgccatttatttccccctggtatctgatgttcatattagtttaatgtgccttttcagagaattcaagacactttttggaaagtagaatttttttttgaaaatttatgattggagaggtactacacaatttagaggttacatttcttgacaaatctgagttgaataaaaaagaactaaaaatataaacatagctaattcaagaatcaagatcgggtgaaactaaattaaaaacagccataaagtcccacattttccctaatttatttacctatgatattggcacatcttgttttacttaacatttgaaaaatacaaatatctcttcatatgcaaaagagcaaatgttaaatgaaaaactgaattttatatagcttcctaaatatgagccacatgcttaagcagtgaattaactttatgaatcaaatgtttaatgttaactattacaaaagcctggtatccaggtgcaatctcaccagaaaaaaatagcacctgcctttattacaataaaaaaaatggctaattccctttgacatcttaagagtgacactactttgtcaagcactaaatactttttaaattaatcatgttaaacttcagatttatagatataaatattgtatttataactttagtcataatgtacaatttctttcttgtttaaaagtactttctcactcaaaatggtatttatagtttaaaaagaatatgcctctgtattcaggagtgattcaaattcccagatgttttcacatagttatgaaaatgggaaagtgctgaattaaactgggctgcaatatttcaagttttttgctatcaggttataaactatacctacgattgcaagtcatacagtgcctctatttctagaaggcttttaaagtttcctggcttagttatgtccaaaggcagcaggaagtctcatcagtagagggcagaattttcaagtgctgccattcttatcccaggaggcatttccagtggttgagcacaaggcctgtttgtagtttgcttttgctcttgcattttgtggaagggaaggaactgagagagcttagagggttcattaaaaccacccctcactctcttagtcgtagtcagatggagtattcataacagtaacctccaattaccactatgtgttgggaaaaattagaattcggtctacttacaatcctgccaactaggattttactttgatatttcagtataacagtgaatctggattgatgcctgattaaaataaaatccctgattattactttctggattacgaactaaaatccctgtaaaatcaatggatgtgactcattgttaagagtcatgcagacttttacatattaggtaagaattctaaaaattatttgagggttctattctctagcaccaggtactaatgctccctactcaaaaaaaatcatgtgcatggattaatcaagtctaacagtgctcagatttaatggtttaacattgattttcttttctttgtcaaacttatatatgcaaatatttttatagtagtcagatgttatttttgaataaggatcaccctcatttttacccatgtgcttatctttaaaaccaacattgtaaagtagcacgcagacatatgtttcttttatcttcatggattatttttaccttaaaaataaattatcatttttttttttgaatttgggttttattctccagatactctgtgtacatgtgggtaagtatgtgggagtatgtgtgtttgtgtgtaagaggggataattaattgtctctcaactctatctcatactttaatatcaaataaaaaatgaaatgtataaagggtcactttgtaggattaggcatcctccttctacctacttaaaccaggggtttgggattcagaattctccatataaccaagaccgaaagtcactggaagactttaaaattagtattttaaccaccacacccagagtcaggtatggaaataaacctatagcatggattctttctatgcataatctcaaaatttaactacccaaataagtaagtttttaaaaactaatttaaaatttgccattgaggaaaatatcacctccatccttaattgtgactcctcatttcagctaaaaccttttctaatactttaaaaaaacaaaatgaaaaacaaactcctagataaagtcataaacactgaaatcagagatgtgattcttgttaaatgttagtttctctttctgaggttacactctgtgcatttgaaactttgacgttaacatcttccgaatgtttagatttgctcaagggttcagattctctggtcttctgccttgcattttcctccttcctttcctttgcaagcaatctatagttgatagcattgccaatgagcagccacacgcttgctgctaccacaatagccccacaggacatgtacatgtatttatattctccagttaaatccaccaatttacctgcaagaggagggccaagaagaactgggccacactccacaattgtgacaagtccgacggcactggaaaatcttggtgcacccacgaggtccatgagagtttcaaagagaacactgctaacactcccaaatccaaggccaaaaaatacagcatataataccaggcttgtgtagtcctgtgccagtgggcacaagaggtgacacactccattgaacatgattgcaaaactgaagaagtactgaattcgaggtcgaatatatttggagtttgcaattaatcctacagaaggcctagcaaacatatcaacgaaagccataacagatagcagaaaagctgccgagtactcatcaattccttggtctttagcatatggagccaagaatataatgggggcaaaaaaacctaggaacataatgacatttccagacagatatatcagaaatcctctatgcttaaaaagggagaaatctaaatacttattaactttttcccaagttgatttcttcgttttgattttctttgggcttgaatcatcttctgttttgccagtcttatttttagacttagaagtggtttgattgggtccaaggggtctcatgagggaaccagccacacaggcattcaaaagtagacttcccaaaatcaggaagcttcctttccagccaaaagtattaaaaaggtactgattgaaaggagccaatgaacttaagaaaacaggacttcctgccatggccaatccatttgccatgggtcgcttcctatagaagtatttgccaattatggttaaggcgggttgcaggttgaaggctaaacctaaacctgtaatgaatcccatagtgaggtacagctgtaccacgctgctactaaaggaggccaacaccattccaagacagcataataagcctcctgctatcaccaccggccggctgccgtatttattcaccaaaacactacttacaggacttcactgaagtcctgagcctcttaaagtcacccatgaggattgaaataaacttcttccaaacttctgttaatgttggtattttgacctcctcccataacagtgaatgatcgtgatgttatctagaatagcaaatcctttccagaagattttccatctccttttcccagattcatcagaggagtcattatgtacggcagctaggcatgatcctgattgagtaaagctgcactgaatcctcaaggatgtgaagatcaaaaagctttcaaatattctacctcctgcgtacataacagccagcataatggatgaaatccatgctatttcactgtaggtagtgtggaatatttgctgaatttctttgaagaatacggtgacagctttggggaatgcataggaaaatccaatggagataaaagctgctccaaccacaatccaaccccatcctccatctggaggtggatgcacaggtggggcacttggcattggtggcatttctgctcctctagtggaaattcaagtaacctggcgacaggtgtttagaaacatggtcttccatttcaccaagacataagtttccctgatctatggactcctctccccacctgaggcagaagtttccttgt

SEQ ID NO: 11057 - RNA, 6518 nt, Homo sapiens
  source 1..6518: mol_type = other RNA
ctgaatagctgggactacaggtgcacatcaccacatccaggtaattattttactttttgaatcatgatatgtagcaaccaatctgggaattatttattcataaaagataacattttcctgctaactccaacctcagaaaaaatgtattatgcctgactcaaatatgtcattatttttatgagaaaaagagtcatattgaagtaattatgtctatatgtaataattatcattatttgagataatttgcattggggagaaaagcaggcaatcagaaattacatattcaaggctgggcgcagtggctcacgcctgtaatcccagcactttgggaggcagaggcgagtgaatcacctgaggtcagagttcaagaccagcctgaccaacaaggagaaaccccatctctactaaaacaaaacaaaacaaaacaaaacaaaaaaagccacaaaattagccgggcatggtggcacatgcctgtaattccagttactcgggaggctgaggcaggagaattgcttgaacctgggaggcagaggttgtagtaagccgagattgtgccactgcacgccagcctgggcgacaagaacgagactcagtctcaaaaaaaaaaaaaaagaaagaaagaaagaaattacatattcaggttctagcaaatgcagttctctaataaacactaaataaatcataatacaagttacagttaaacctaattgttttactatataggatgtatcttttttgtacctatattttatcttcctttgcttctctggcctctattgggaggcagcacggtagtgaacacctcggggatctttctggttacgtaaacctgagttttaattttggttcatactaccttttaactttgggtagtctgctgagcttgttttttgttttcactcatctgtcatatcaagctagtaataattctgccatggttttggttttcatattgaaaggcattacataagcaaaatgcataacatataaatattagttccctttccactatgcatccaatctccctattaaattaagcctaaaaataataatttttgttttattaaaagccttccacattctacatatgaaagggattttttaaaggtgttttagataaaaaatgtttcaaccaactgaccaagaatatctcttcatatttatgtcatctacataaaaacttacatttatatcatatatcttttagtcttcttttctatattcttgattgtcatgttgtacagccagaaaagaatgagtataaattatctagattttttaaagtgcacattcaaacatagaaaatctaattattttacttgtttcttagtattaggctgaggccaatgagtccatgagctaaagggttgaaacttggcaccaaaaaagtgattgtttatgagtcctgtagatttatactgagaaaacatcatgtcttccaatgtgaaatacactaaaacctgattttttgtctcttaaggtgtgctaggtgaatgcaaaaaggatcaggaaagggggtgaggataggtcaggaaaagtgcaaacacaatgttctattcataaattagtgatggcatatttaaggttaagtagtaaaaaatatggggggctcagttaacacgaatgaaaaaatagttaaagtagccatgaattatctggataccttgatttaatgacaccctttcttctgtacaatttcataatgtgggaatagagattagtggggattgtagtggtataccctgactttgcttcatgatatctcaaatgtttaaaacctattattccctagagaaagaaatatgttcatactaattgttgcagaggcagaagccaaatatatctcctcctccatttatgtgactatatagtaatgaaaatcctaggttgatacacttttctcaatcttggaaagattctgctaaagcagcaaatcttctaacaagttcaagagggtggggagagtgaacaagtagaataatttatattaccctggaacaattctgaatcctgtaggtatttatgtcactgtttcaattgtgttctggtttaactgtcaatatttatgcatagcagttaacgtgtgtgcatatttgtaactgtgcagtgctactgccaggtgtgactgtacaaatcatgtgctttgaatgtgcaagttttactttcttttctaacaatttaatacagtgttagaaataaataacgaatgaagacaaccaaagagcagccagacaaatgtgaactggttttgacgtgacgagaaactcatcagtaagtaaataaacctcctccctggagaaggccactgaaatgcacccaggaggatgtctctactagaaggtaataaaaaatatatataatgtagtctttgacctaaaacctcatgattattactttgccatttatttccccctggtatctgatgttcatattagtttaatgtgccttttcagagaattcaagacactttttggaaagtagaatttttttttgaaaatttatgattggagaggtactacacaatttagaggttacatttcttgacaaatctgagttgaataaaaaagaactaaaaatataaacatagctaattcaagaatcaagatcgggtgaaactaaattaaaaacagccataaagtcccacattttccctaatttatttacctatgatattggcacatcttgttttacttaacatttgaaaaatacaaatatctcttcatatgcaaaagagcaaatgttaaatgaaaaactgaattttatatagcttcctaaatatgagccacatgcttaagcagtgaattaactttatgaatcaaatgtttaatgttaactattacaaaagcctggtatccaggtgcaatctcaccagaaaaaaatagcacctgcctttattacaataaaaaaaatggctaattccctttgacatcttaagagtgacactactttgtcaagcactaaatactttttaaattaatcatgttaaacttcagatttatagatataaatattgtatttataactttagtcataatgtacaatttctttcttgtttaaaagtactttctcactcaaaatggtatttatagtttaaaaagaatatgcctctgtattcaggagtgattcaaattcccagatgttttcacatagttatgaaaatgggaaagtgctgaattaaactgggctgcaatatttcaagttttttgctatcaggttataaactatacctacgattgcaagtcatacagtgcctctatttctagaaggcttttaaagtttcctggcttagttatgtccaaaggcagcaggaagtctcatcagtagagggcagaattttcaagtgctgccattcttatcccaggaggcatttccagtggttgagcacaaggcctgtttgtagtttgcttttgctcttgcattttgtggaagggaaggaactgagagagcttagagggttcattaaaaccacccctcactctcttagtcgtagtcagatggagtattcataacagtaacctccaattaccactatgtgttgggaaaaattagaattcggtctacttacaatcctgccaactaggattttactttgatatttcagtataacagtgaatctggattgatgcctgattaaaataaaatccctgattattactttctggattacgaactaaaatccctgtaaaatcaatggatgtgactcattgttaagagtcatgcagacttttacatattaggtaagaattctaaaaattatttgagggttctattctctagcaccaggtactaatgctccctactcaaaaaaaatcatgtgcatggattaatcaagtctaacagtgctcagatttaatggtttaacattgattttcttttctttgtcaaacttatatatgcaaatatttttatagtagtcagatgttatttttgaataaggatcaccctcatttttacccatgtgcttatctttaaaaccaacattgtaaagtagcacgcagacatatgtttcttttatcttcatggattatttttaccttaaaaataaattatcatttttttttttgaatttgggttttattctccagatactctgtgtacatgtgggtaagtatgtgggagtatgtgtgtttgtgtgtaagaggggataattaattgtctctcaactctatctcatactttaatatcaaataaaaaatgaaatgtataaagggtcactttgtaggattaggcatcctccttctacctacttaaaccaggggtttgggattcagaattctccatataaccaagaccgaaagtcactggaagactttaaaattagtattttaaccaccacacccagagtcaggtatggaaataaacctatagcatggattctttctatgcataatctcaaaatttaactacccaaataagtaagtttttaaaaactaatttaaaatttgccattgaggaaaatatcacctccatccttaattgtgactcctcatttcagctaaaaccttttctaatactttaaaaaaacaaaatgaaaaacaaactcctagataaagtcataaacactgaaatcagagatgtgattcttgttaaatgttagtttctctttctgaggttacactctgtgcatttgaaactttgacgttaacatcttccgaatgtttagatttgctcaagggttcagattctctggtcttctgccttgcattttcctccttcctttcctttgcaagcaatctatagttgatagcattgccaatgagcagccacacgcttgctgctaccacaatagccccacaggacatgtacatgtatttatattctccagttaaatccaccaatttacctgcaagaggagggccaagaagaactgggccacactccacaattgtgacaagtccgacggcactggaaaatcttggtgcacccacgaggtccatgagagtttcaaagagaacactgctaacactcccaaatccaaggccaaaaaatacagcatataataccaggcttgtgtagtcctgtgccagtgggcacaagaggtgacacactccattgaacatgattgcaaaactgaagaagtactgaattcgaggtcgaatatatttggagtttgcaattaatcctacagaaggcctagcaaacatatcaacgaaagccataacagatagcagaaaagctgccgagtactcatcaattccttggtctttagcatatggagccaagaatataatgggggcaaaaaaacctaggaacataatgacatttccagacagatatatcagaaatcctctatgcttaaaaagggagaaatctaaatacttattaactttttcccaagttgatttcttcgttttgattttctttgggcttgaatcatcttctgttttgccagtcttatttttagacttagaagtggtttgattgggtccaaggggtctcatgagggaaccagccacacaggcattcaaaagtagacttcccaaaatcaggaagcttcctttccagccaaaagtattaaaaaggtactgattgaaaggagccaatgaacttaagaaaacaggacttcctgccatggccaatccatttgccatgggtcgcttcctatagaagtatttgccaattatggttaaggcgggttgcaggttgaaggctaaacctaaacctgtaatgaatcccatagtgaggtacagctgtaccacgctgctactaaaggaggccaacaccattccaagacagcataataagcctcctgctatcaccaccggccggctgccgtatttattcaccaaaacactacttacaggacttcactgaagtcctgagcctcttaaagtcacccatgaggattgaaataaacttcttccaaacttctgttaatgttggtattttgacctcctcccataacagtgaatgatcgtgatgttatctagaatagcaaatcctttccagaagattttccatctccttttcccagattcatcagaggagtcattatgtacggcagctgtaagctaggcatgatcctgattgagtaaagctgcactgaatcctcaaggatgtgaagatcaaaaagctttcaaatattctacctcaagtagatggtgatctctttaaagggtgaatgatgcattccgcttctccttttttcctcctgcgtacataacagccagcataatggatgaaatccatgctatttcactgtaggtagtgtggaatatttgctgaatttctttgaagaatacggtgacagctttggggaatgcataggaaaatccaatggagataaaagctgctccaaccacaatccaaccccatcctccatctggaggtggatgcacaggtggggcacttggcattggtggcatttctgctcctctagtggaaattcaagtaacctggcgacaggtgtttagaaacatggtcttccatttcaccaagacataagtttccctgatctatggactcctctccccacctgaggcagaagtttccttgtgaaccattgctctttttagaat

SEQ ID NO: 11058 - RNA, 6844 nt, Homo sapiens
  source 1..6844: mol_type = other RNA
ctgaatagctgggactacaggtgcacatcaccacatccaggtaattattttactttttgaatcatgatatgtagcaaccaatctgggaattatttattcataaaagataacattttcctgctaactccaacctcagaaaaaatgtattatgcctgactcaaatatgtcattatttttatgagaaaaagagtcatattgaagtaattatgtctatatgtaataattatcattatttgagataatttgcattggggagaaaagcaggcaatcagaaattacatattcaaggctgggcgcagtggctcacgcctgtaatcccagcactttgggaggcagaggcgagtgaatcacctgaggtcagagttcaagaccagcctgaccaacaaggagaaaccccatctctactaaaacaaaacaaaacaaaacaaaacaaaaaaagccacaaaattagccgggcatggtggcacatgcctgtaattccagttactcgggaggctgaggcaggagaattgcttgaacctgggaggcagaggttgtagtaagccgagattgtgccactgcacgccagcctgggcgacaagaacgagactcagtctcaaaaaaaaaaaaaaagaaagaaagaaagaaattacatattcaggttctagcaaatgcagttctctaataaacactaaataaatcataatacaagttacagttaaacctaattgttttactatataggatgtatcttttttgtacctatattttatcttcctttgcttctctggcctctattgggaggcagcacggtagtgaacacctcggggatctttctggttacgtaaacctgagttttaattttggttcatactaccttttaactttgggtagtctgctgagcttgttttttgttttcactcatctgtcatatcaagctagtaataattctgccatggttttggttttcatattgaaaggcattacataagcaaaatgcataacatataaatattagttccctttccactatgcatccaatctccctattaaattaagcctaaaaataataatttttgttttattaaaagccttccacattctacatatgaaagggattttttaaaggtgttttagataaaaaatgtttcaaccaactgaccaagaatatctcttcatatttatgtcatctacataaaaacttacatttatatcatatatcttttagtcttcttttctatattcttgattgtcatgttgtacagccagaaaagaatgagtataaattatctagattttttaaagtgcacattcaaacatagaaaatctaattattttacttgtttcttagtattaggctgaggccaatgagtccatgagctaaagggttgaaacttggcaccaaaaaagtgattgtttatgagtcctgtagatttatactgagaaaacatcatgtcttccaatgtgaaatacactaaaacctgattttttgtctcttaaggtgtgctaggtgaatgcaaaaaggatcaggaaagggggtgaggataggtcaggaaaagtgcaaacacaatgttctattcataaattagtgatggcatatttaaggttaagtagtaaaaaatatggggggctcagttaacacgaatgaaaaaatagttaaagtagccatgaattatctggataccttgatttaatgacaccctttcttctgtacaatttcataatgtgggaatagagattagtggggattgtagtggtataccctgactttgcttcatgatatctcaaatgtttaaaacctattattccctagagaaagaaatatgttcatactaattgttgcagaggcagaagccaaatatatctcctcctccatttatgtgactatatagtaatgaaaatcctaggttgatacacttttctcaatcttggaaagattctgctaaagcagcaaatcttctaacaagttcaagagggtggggagagtgaacaagtagaataatttatattaccctggaacaattctgaatcctgtaggtatttatgtcactgtttcaattgtgttctggtttaactgtcaatatttatgcatagcagttaacgtgtgtgcatatttgtaactgtgcagtgctactgccaggtgtgactgtacaaatcatgtgctttgaatgtgcaagttttactttcttttctaacaatttaatacagtgttagaaataaataacgaatgaagacaaccaaagagcagccagacaaatgtgaactggttttgacgtgacgagaaactcatcagtaagtaaataaacctcctccctggagaaggccactgaaatgcacccaggaggatgtctctactagaaggtaataaaaaatatatataatgtagtctttgacctaaaacctcatgattattactttgccatttatttccccctggtatctgatgttcatattagtttaatgtgccttttcagagaattcaagacactttttggaaagtagaatttttttttgaaaatttatgattggagaggtactacacaatttagaggttacatttcttgacaaatctgagttgaataaaaaagaactaaaaatataaacatagctaattcaagaatcaagatcgggtgaaactaaattaaaaacagccataaagtcccacattttccctaatttatttacctatgatattggcacatcttgttttacttaacatttgaaaaatacaaatatctcttcatatgcaaaagagcaaatgttaaatgaaaaactgaattttatatagcttcctaaatatgagccacatgcttaagcagtgaattaactttatgaatcaaatgtttaatgttaactattacaaaagcctggtatccaggtgcaatctcaccagaaaaaaatagcacctgcctttattacaataaaaaaaatggctaattccctttgacatcttaagagtgacactactttgtcaagcactaaatactttttaaattaatcatgttaaacttcagatttatagatataaatattgtatttataactttagtcataatgtacaatttctttcttgtttaaaagtactttctcactcaaaatggtatttatagtttaaaaagaatatgcctctgtattcaggagtgattcaaattcccagatgttttcacatagttatgaaaatgggaaagtgctgaattaaactgggctgcaatatttcaagttttttgctatcaggttataaactatacctacgattgcaagtcatacagtgcctctatttctagaaggcttttaaagtttcctggcttagttatgtccaaaggcagcaggaagtctcatcagtagagggcagaattttcaagtgctgccattcttatcccaggaggcatttccagtggttgagcacaaggcctgtttgtagtttgcttttgctcttgcattttgtggaagggaaggaactgagagagcttagagggttcattaaaaccacccctcactctcttagtcgtagtcagatggagtattcataacagtaacctccaattaccactatgtgttgggaaaaattagaattcggtctacttacaatcctgccaactaggattttactttgatatttcagtataacagtgaatctggattgatgcctgattaaaataaaatccctgattattactttctggattacgaactaaaatccctgtaaaatcaatggatgtgactcattgttaagagtcatgcagacttttacatattaggtaagaattctaaaaattatttgagggttctattctctagcaccaggtactaatgctccctactcaaaaaaaatcatgtgcatggattaatcaagtctaacagtgctcagatttaatggtttaacattgattttcttttctttgtcaaacttatatatgcaaatatttttatagtagtcagatgttatttttgaataaggatcaccctcatttttacccatgtgcttatctttaaaaccaacattgtaaagtagcacgcagacatatgtttcttttatcttcatggattatttttaccttaaaaataaattatcatttttttttttgaatttgggttttattctccagatactctgtgtacatgtgggtaagtatgtgggagtatgtgtgtttgtgtgtaagaggggataattaattgtctctcaactctatctcatactttaatatcaaataaaaaatgaaatgtataaagggtcactttgtaggattaggcatcctccttctacctacttaaaccaggggtttgggattcagaattctccatataaccaagaccgaaagtcactggaagactttaaaattagtattttaaccaccacacccagagtcaggtatggaaataaacctatagcatggattctttctatgcataatctcaaaatttaactacccaaataagtaagtttttaaaaactaatttaaaatttgccattgaggaaaatatcacctccatccttaattgtgactcctcatttcagctaaaaccttttctaatactttaaaaaaacaaaatgaaaaacaaactcctagataaagtcataaacactgaaatcagagatgtgattcttgttaaatgttagtttctctttctgaggttacactctgtgcatttgaaactttgacgttaacatcttccgaatgtttagatttgctcaagggttcagattctctggtcttctgccttgcattttcctccttcctttcctttgcaagcaatctatagttgatagcattgccaatgagcagccacacgcttgctgctaccacaatagccccacaggacatgtacatgtatttatattctccagttaaatccaccaatttacctgcaagaggagggccaagaagaactgggccacactccacaattgtgacaagtccgacggcactggaaaatcttggtgcacccacgaggtccatgagagtttcaaagagaacactgctaacactcccaaatccaaggccaaaaaatacagcatataataccaggcttgtgtagtcctgtgccagtgggcacaagaggtgacacactccattgaacatgattgcaaaactgaagaagtactgaattcgaggtcgaatatatttggagtttgcaattaatcctacagaaggcctagcaaacatatcaacgaaagccataacagatagcagaaaagctgccgagtactcatcaattccttggtctttagcatatggagccaagaatataatgggggcaaaaaaacctaggaacataatgacatttccagacagatatatcagaaatcctctatgcttaaaaagggagaaatctaaatacttattaactttttcccaagttgatttcttcgttttgattttctttgggcttgaatcatcttctgttttgccagtcttatttttagacttagaagtggtttgattgggtccaaggggtctcatgagggaaccagccacacaggcattcaaaagtagacttcccaaaatcaggaagcttcctttccagccaaaagtattaaaaaggtactgattgaaaggagccaatgaacttaagaaaacaggacttcctgccatggccaatccatttgccatgggtcgcttcctatagaagtatttgccaattatggttaaggcgggttgcaggttgaaggctaaacctaaacctgtaatgaatcccatagtgaggtacagctgtaccacgctgctactaaaggaggccaacaccattccaagacagcataataagcctcctgctatcaccaccggccggctgccgtatttattcaccaaaacactacttacaggacttcactgaagtcctgagcctcttaaagtcacccatgaggattgaaataaacttcttccaaacttctgttaatgttggtattttgacctcctcccataacagtgaatgatcgtgatgttatctagaatagcaaatcctttccagaagattttccatctccttttcccagattcatcagaggagtcattatgtacggcagctgtaagcttcagtagaattgaagacagttagggccctgctctggattaggctctggcttagggaatgttgtgggtggtttgatcttgtatccaaacttctaaaactttcttcacttttcctttgcattcacaacttggctaaccttagtgctagacacctagctttcagcctgtgctttcagcacctttctcattaaggtgaatcatttctagcttttgatttcaaatgagagacttgcaactcttcctttcacttgaacacttagaagccactgtaggtttattaagtggcctaatttcaatactgttgtatctcagacagtagagaggccctaggcatgatcctgattgagtaaagctgcactgaatcctcaaggatgtgaagatcaaaaagctttcaaatattctacctcaagtagatggtgatctctttaaagggtgaatgatgcattccgcttctccttttttcctcctgcgtacataacagccagcataatggatgaaatccatgctatttcactgtaggtagtgtggaatatttgctgaatttctttgaagaatacggtgacagctttggggaatgcataggaaaatccaatggagataaaagctgctccaaccacaatccaaccccatcctccatctggaggtggatgcacaggtggggcacttggcattggtggcatttctgctcctctagtggaaattcaagtaacctggcgacaggtgtttagaaacatggtcttccatttcaccaagacataagtttccctgatctatggactcctctccccacctgaggcagaagtttccttgtgaaccattgctctttttagaat

SEQ ID NO: 11059 - RNA, 6918 nt, Homo sapiens
  source 1..6918: mol_type = other RNA
ctgaatagctgggactacaggtgcacatcaccacatccaggtaattattttactttttgaatcatgatatgtagcaaccaatctgggaattatttattcataaaagataacattttcctgctaactccaacctcagaaaaaatgtattatgcctgactcaaatatgtcattatttttatgagaaaaagagtcatattgaagtaattatgtctatatgtaataattatcattatttgagataatttgcattggggagaaaagcaggcaatcagaaattacatattcaaggctgggcgcagtggctcacgcctgtaatcccagcactttgggaggcagaggcgagtgaatcacctgaggtcagagttcaagaccagcctgaccaacaaggagaaaccccatctctactaaaacaaaacaaaacaaaacaaaacaaaaaaagccacaaaattagccgggcatggtggcacatgcctgtaattccagttactcgggaggctgaggcaggagaattgcttgaacctgggaggcagaggttgtagtaagccgagattgtgccactgcacgccagcctgggcgacaagaacgagactcagtctcaaaaaaaaaaaaaaagaaagaaagaaagaaattacatattcaggttctagcaaatgcagttctctaataaacactaaataaatcataatacaagttacagttaaacctaattgttttactatataggatgtatcttttttgtacctatattttatcttcctttgcttctctggcctctattgggaggcagcacggtagtgaacacctcggggatctttctggttacgtaaacctgagttttaattttggttcatactaccttttaactttgggtagtctgctgagcttgttttttgttttcactcatctgtcatatcaagctagtaataattctgccatggttttggttttcatattgaaaggcattacataagcaaaatgcataacatataaatattagttccctttccactatgcatccaatctccctattaaattaagcctaaaaataataatttttgttttattaaaagccttccacattctacatatgaaagggattttttaaaggtgttttagataaaaaatgtttcaaccaactgaccaagaatatctcttcatatttatgtcatctacataaaaacttacatttatatcatatatcttttagtcttcttttctatattcttgattgtcatgttgtacagccagaaaagaatgagtataaattatctagattttttaaagtgcacattcaaacatagaaaatctaattattttacttgtttcttagtattaggctgaggccaatgagtccatgagctaaagggttgaaacttggcaccaaaaaagtgattgtttatgagtcctgtagatttatactgagaaaacatcatgtcttccaatgtgaaatacactaaaacctgattttttgtctcttaaggtgtgctaggtgaatgcaaaaaggatcaggaaagggggtgaggataggtcaggaaaagtgcaaacacaatgttctattcataaattagtgatggcatatttaaggttaagtagtaaaaaatatggggggctcagttaacacgaatgaaaaaatagttaaagtagccatgaattatctggataccttgatttaatgacaccctttcttctgtacaatttcataatgtgggaatagagattagtggggattgtagtggtataccctgactttgcttcatgatatctcaaatgtttaaaacctattattccctagagaaagaaatatgttcatactaattgttgcagaggcagaagccaaatatatctcctcctccatttatgtgactatatagtaatgaaaatcctaggttgatacacttttctcaatcttggaaagattctgctaaagcagcaaatcttctaacaagttcaagagggtggggagagtgaacaagtagaataatttatattaccctggaacaattctgaatcctgtaggtatttatgtcactgtttcaattgtgttctggtttaactgtcaatatttatgcatagcagttaacgtgtgtgcatatttgtaactgtgcagtgctactgccaggtgtgactgtacaaatcatgtgctttgaatgtgcaagttttactttcttttctaacaatttaatacagtgttagaaataaataacgaatgaagacaaccaaagagcagccagacaaatgtgaactggttttgacgtgacgagaaactcatcagtaagtaaataaacctcctccctggagaaggccactgaaatgcacccaggaggatgtctctactagaaggtaataaaaaatatatataatgtagtctttgacctaaaacctcatgattattactttgccatttatttccccctggtatctgatgttcatattagtttaatgtgccttttcagagaattcaagacactttttggaaagtagaatttttttttgaaaatttatgattggagaggtactacacaatttagaggttacatttcttgacaaatctgagttgaataaaaaagaactaaaaatataaacatagctaattcaagaatcaagatcgggtgaaactaaattaaaaacagccataaagtcccacattttccctaatttatttacctatgatattggcacatcttgttttacttaacatttgaaaaatacaaatatctcttcatatgcaaaagagcaaatgttaaatgaaaaactgaattttatatagcttcctaaatatgagccacatgcttaagcagtgaattaactttatgaatcaaatgtttaatgttaactattacaaaagcctggtatccaggtgcaatctcaccagaaaaaaatagcacctgcctttattacaataaaaaaaatggctaattccctttgacatcttaagagtgacactactttgtcaagcactaaatactttttaaattaatcatgttaaacttcagatttatagatataaatattgtatttataactttagtcataatgtacaatttctttcttgtttaaaagtactttctcactcaaaatggtatttatagtttaaaaagaatatgcctctgtattcaggagtgattcaaattcccagatgttttcacatagttatgaaaatgggaaagtgctgaattaaactgggctgcaatatttcaagttttttgctatcaggttataaactatacctacgattgcaagtcatacagtgcctctatttctagaaggcttttaaagtttcctggcttagttatgtccaaaggcagcaggaagtctcatcagtagagggcagaattttcaagtgctgccattcttatcccaggaggcatttccagtggttgagcacaaggcctgtttgtagtttgcttttgctcttgcattttgtggaagggaaggaactgagagagcttagagggttcattaaaaccacccctcactctcttagtcgtagtcagatggagtattcataacagtaacctccaattaccactatgtgttgggaaaaattagaattcggtctacttacaatcctgccaactaggattttactttgatatttcagtataacagtgaatctggattgatgcctgattaaaataaaatccctgattattactttctggattacgaactaaaatccctgtaaaatcaatggatgtgactcattgttaagagtcatgcagacttttacatattaggtaagaattctaaaaattatttgagggttctattctctagcaccaggtactaatgctccctactcaaaaaaaatcatgtgcatggattaatcaagtctaacagtgctcagatttaatggtttaacattgattttcttttctttgtcaaacttatatatgcaaatatttttatagtagtcagatgttatttttgaataaggatcaccctcatttttacccatgtgcttatctttaaaaccaacattgtaaagtagcacgcagacatatgtttcttttatcttcatggattatttttaccttaaaaataaattatcatttttttttttgaatttgggttttattctccagatactctgtgtacatgtgggtaagtatgtgggagtatgtgtgtttgtgtgtaagaggggataattaattgtctctcaactctatctcatactttaatatcaaataaaaaatgaaatgtataaagggtcactttgtaggattaggcatcctccttctacctacttaaaccaggggtttgggattcagaattctccatataaccaagaccgaaagtcactggaagactttaaaattagtattttaaccaccacacccagagtcaggtatggaaataaacctatagcatggattctttctatgcataatctcaaaatttaactacccaaataagtaagtttttaaaaactaatttaaaatttgccattgaggaaaatatcacctccatccttaattgtgactcctcatttcagctaaaaccttttctaatactttaaaaaaacaaaatgaaaaacaaactcctagataaagtcataaacactgaaatcagagatgtgattcttgttaaatgttagtttctctttctgaggttacactctgtgcatttgaaactttgacgttaacatcttccgaatgtttagatttgctcaagggttcagattctctggtcttctgccttgcattttcctccttcctttcctttgcaagcaatctatagttgatagcattgccaatgagcagccacacgcttgctgctaccacaatagccccacaggacatgtacatgtatttatattctccagttaaatccaccaatttacctgcaagaggagggccaagaagaactgggccacactccacaattgtgacaagtccgacggcactggaaaatcttggtgcacccacgaggtccatgagagtttcaaagagaacactgctaacactcccaaatccaaggccaaaaaatacagcatataataccaggcttgtgtagtcctgtgccagtgggcacaagaggtgacacactccattgaacatgattgcaaaactgaagaagtactgaattcgaggtcgaatatatttggagtttgcaattaatcctacagaaggcctagcaaacatatcaacgaaagccataacagatagcagaaaagctgccgagtactcatcaattccttggtctttagcatatggagccaagaatataatgggggcaaaaaaacctaggaacataatgacatttccagacagatatatcagaaatcctctatgcttaaaaagggagaaatctaaatacttattaactttttcccaagttgatttcttcgttttgattttctttgggcttgaatcatcttctgttttgccagtcttatttttagacttagaagtggtttgattgggtccaaggggtctcatgagggaaccagccacacaggcattcaaaagtagacttcccaaaatcaggaagcttcctttccagccaaaagtattaaaaaggtactgattgaaaggagccaatgaacttaagaaaacaggacttcctgccatggccaatccatttgccatgggtcgcttcctatagaagtatttgccaattatggttaaggcgggttgcaggttgaaggctaaacctaaacctgtaatgaatcccatagtgaggtacagctgtaccacgctgctactaaaggaggccaacaccattccaagacagcataataagcctcctgctatcaccaccggccggctgccgtatttattcaccaaaacactacttacaggacttcactgaagtcctgagcctcttaaagtcacccatgaggattgaaataaacttcttccaaacttctgttaatgttggtattttgacctcctcccataacagtgaatgatcgtgatgttatctagaatagcaaatcctttccagaagattttccatctccttttcccagattcatcagaggagtcattatgtacggcagctgtaagcttcagtagaattgaagacagttagggccctgctctggattaggctctggcttagggaatgttgtgggtggtttgatcttgtatccaaacttctaaaactttcttcacttttcctttgcattcacaacttggctaaccttagtgctagacacctagctttcagcctgtgctttcagcacctttctcattaaggtgaatcatttctagcttttgatttcaaatgagagacttgcaactcttcctttcacttgaacacttagaagccactgtaggtttattaagtggcctaatttcaatactgttgtatctcagacagtagagaggccctaggcatgatcctgattgagtaaagctgcactgaatcctcaaggatgtgaagatcaaaaagctttcaaatattctacctcaagtagatggtgatctctttaaagggtgaatgatgcattccgcttctccttttttcctgggtgccatggagggcatgttgatggtgggaggcagacagattcctgggcagaaaggggtggatccttggtgaaaccccacctttaatccagagacagcctgaggcctgggggtcagactgtcagttctgggtagtctgtagaccaaagtgagaacttatggagctttttccaggcccacccatggctgcccacagaccaatcagcatgcacttcctcccttctgaccccttaaaaaccccagactctgccagactcacacagacgtcaggattaccagctgtgggaaggagatacccactttgggtctcctcagctagtcaggacgacctgcctgcagaaagaaggtgcccaccgtggctctcctaagagttgttttgttgctcagtgaagctcctctctgccttgctcgctctccggttgtccatgtgcttcattcttcc

SEQ ID NO: 11060 - RNA, 6973 nt, Homo sapiens
  source 1..6973: mol_type = other RNA
ctgaatagctgggactacaggtgcacatcaccacatccaggtaattattttactttttgaatcatgatatgtagcaaccaatctgggaattatttattcataaaagataacattttcctgctaactccaacctcagaaaaaatgtattatgcctgactcaaatatgtcattatttttatgagaaaaagagtcatattgaagtaattatgtctatatgtaataattatcattatttgagataatttgcattggggagaaaagcaggcaatcagaaattacatattcaaggctgggcgcagtggctcacgcctgtaatcccagcactttgggaggcagaggcgagtgaatcacctgaggtcagagttcaagaccagcctgaccaacaaggagaaaccccatctctactaaaacaaaacaaaacaaaacaaaacaaaaaaagccacaaaattagccgggcatggtggcacatgcctgtaattccagttactcgggaggctgaggcaggagaattgcttgaacctgggaggcagaggttgtagtaagccgagattgtgccactgcacgccagcctgggcgacaagaacgagactcagtctcaaaaaaaaaaaaaaagaaagaaagaaagaaattacatattcaggttctagcaaatgcagttctctaataaacactaaataaatcataatacaagttacagttaaacctaattgttttactatataggatgtatcttttttgtacctatattttatcttcctttgcttctctggcctctattgggaggcagcacggtagtgaacacctcggggatctttctggttacgtaaacctgagttttaattttggttcatactaccttttaactttgggtagtctgctgagcttgttttttgttttcactcatctgtcatatcaagctagtaataattctgccatggttttggttttcatattgaaaggcattacataagcaaaatgcataacatataaatattagttccctttccactatgcatccaatctccctattaaattaagcctaaaaataataatttttgttttattaaaagccttccacattctacatatgaaagggattttttaaaggtgttttagataaaaaatgtttcaaccaactgaccaagaatatctcttcatatttatgtcatctacataaaaacttacatttatatcatatatcttttagtcttcttttctatattcttgattgtcatgttgtacagccagaaaagaatgagtataaattatctagattttttaaagtgcacattcaaacatagaaaatctaattattttacttgtttcttagtattaggctgaggccaatgagtccatgagctaaagggttgaaacttggcaccaaaaaagtgattgtttatgagtcctgtagatttatactgagaaaacatcatgtcttccaatgtgaaatacactaaaacctgattttttgtctcttaaggtgtgctaggtgaatgcaaaaaggatcaggaaagggggtgaggataggtcaggaaaagtgcaaacacaatgttctattcataaattagtgatggcatatttaaggttaagtagtaaaaaatatggggggctcagttaacacgaatgaaaaaatagttaaagtagccatgaattatctggataccttgatttaatgacaccctttcttctgtacaatttcataatgtgggaatagagattagtggggattgtagtggtataccctgactttgcttcatgatatctcaaatgtttaaaacctattattccctagagaaagaaatatgttcatactaattgttgcagaggcagaagccaaatatatctcctcctccatttatgtgactatatagtaatgaaaatcctaggttgatacacttttctcaatcttggaaagattctgctaaagcagcaaatcttctaacaagttcaagagggtggggagagtgaacaagtagaataatttatattaccctggaacaattctgaatcctgtaggtatttatgtcactgtttcaattgtgttctggtttaactgtcaatatttatgcatagcagttaacgtgtgtgcatatttgtaactgtgcagtgctactgccaggtgtgactgtacaaatcatgtgctttgaatgtgcaagttttactttcttttctaacaatttaatacagtgttagaaataaataacgaatgaagacaaccaaagagcagccagacaaatgtgaactggttttgacgtgacgagaaactcatcagtaagtaaataaacctcctccctggagaaggccactgaaatgcacccaggaggatgtctctactagaaggtaataaaaaatatatataatgtagtctttgacctaaaacctcatgattattactttgccatttatttccccctggtatctgatgttcatattagtttaatgtgccttttcagagaattcaagacactttttggaaagtagaatttttttttgaaaatttatgattggagaggtactacacaatttagaggttacatttcttgacaaatctgagttgaataaaaaagaactaaaaatataaacatagctaattcaagaatcaagatcgggtgaaactaaattaaaaacagccataaagtcccacattttccctaatttatttacctatgatattggcacatcttgttttacttaacatttgaaaaatacaaatatctcttcatatgcaaaagagcaaatgttaaatgaaaaactgaattttatatagcttcctaaatatgagccacatgcttaagcagtgaattaactttatgaatcaaatgtttaatgttaactattacaaaagcctggtatccaggtgcaatctcaccagaaaaaaatagcacctgcctttattacaataaaaaaaatggctaattccctttgacatcttaagagtgacactactttgtcaagcactaaatactttttaaattaatcatgttaaacttcagatttatagatataaatattgtatttataactttagtcataatgtacaatttctttcttgtttaaaagtactttctcactcaaaatggtatttatagtttaaaaagaatatgcctctgtattcaggagtgattcaaattcccagatgttttcacatagttatgaaaatgggaaagtgctgaattaaactgggctgcaatatttcaagttttttgctatcaggttataaactatacctacgattgcaagtcatacagtgcctctatttctagaaggcttttaaagtttcctggcttagttatgtccaaaggcagcaggaagtctcatcagtagagggcagaattttcaagtgctgccattcttatcccaggaggcatttccagtggttgagcacaaggcctgtttgtagtttgcttttgctcttgcattttgtggaagggaaggaactgagagagcttagagggttcattaaaaccacccctcactctcttagtcgtagtcagatggagtattcataacagtaacctccaattaccactatgtgttgggaaaaattagaattcggtctacttacaatcctgccaactaggattttactttgatatttcagtataacagtgaatctggattgatgcctgattaaaataaaatccctgattattactttctggattacgaactaaaatccctgtaaaatcaatggatgtgactcattgttaagagtcatgcagacttttacatattaggtaagaattctaaaaattatttgagggttctattctctagcaccaggtactaatgctccctactcaaaaaaaatcatgtgcatggattaatcaagtctaacagtgctcagatttaatggtttaacattgattttcttttctttgtcaaacttatatatgcaaatatttttatagtagtcagatgttatttttgaataaggatcaccctcatttttacccatgtgcttatctttaaaaccaacattgtaaagtagcacgcagacatatgtttcttttatcttcatggattatttttaccttaaaaataaattatcatttttttttttgaatttgggttttattctccagatactctgtgtacatgtgggtaagtatgtgggagtatgtgtgtttgtgtgtaagaggggataattaattgtctctcaactctatctcatactttaatatcaaataaaaaatgaaatgtataaagggtcactttgtaggattaggcatcctccttctacctacttaaaccaggggtttgggattcagaattctccatataaccaagaccgaaagtcactggaagactttaaaattagtattttaaccaccacacccagagtcaggtatggaaataaacctatagcatggattctttctatgcataatctcaaaatttaactacccaaataagtaagtttttaaaaactaatttaaaatttgccattgaggaaaatatcacctccatccttaattgtgactcctcatttcagctaaaaccttttctaatactttaaaaaaacaaaatgaaaaacaaactcctagataaagtcataaacactgaaatcagagatgtgattcttgttaaatgttagtttctctttctgaggttacactctgtgcatttgaaactttgacgttaacatcttccgaatgtttagatttgctcaagggttcagattctctggtcttctgccttgcattttcctccttcctttcctttgcaagcaatctatagttgatagcattgccaatgagcagccacacgcttgctgctaccacaatagccccacaggacatgtacatgtatttatattctccagttaaatccaccaatttacctgcaagaggagggccaagaagaactgggccacactccacaattgtgacaagtccgacggcactggaaaatcttggtgcacccacgaggtccatgagagtttcaaagagaacactgctaacactcccaaatccaaggccaaaaaatacagcatataataccaggcttgtgtagtcctgtgccagtgggcacaagaggtgacacactccattgaacatgattgcaaaactgaagaagtactgaattcgaggtcgaatatatttggagtttgcaattaatcctacagaaggcctagcaaacatatcaacgaaagccataacagatagcagaaaagctgccgagtactcatcaattccttggtctttagcatatggagccaagaatataatgggggcaaaaaaacctaggaacataatgacatttccagacagatatatcagaaatcctctatgcttaaaaagggagaaatctaaatacttattaactttttcccaagttgatttcttcgttttgattttctttgggcttgaatcatcttctgttttgccagtcttatttttagacttagaagtggtttgattgggtccaaggggtctcatgagggaaccagccacacaggcattcaaaagtagacttcccaaaatcaggaagcttcctttccagccaaaagtattaaaaaggtactgattgaaaggagccaatgaacttaagaaaacaggacttcctgccatggccaatccatttgccatgggtcgcttcctatagaagtatttgccaattatggttaaggcgggttgcaggttgaaggctaaacctaaacctgtaatgaatcccatagtgaggtacagctgtaccacgctgctactaaaggaggccaacaccattccaagacagcataataagcctcctgctatcaccaccggccggctgccgtatttattcaccaaaacactacttacaggacttcactgaagtcctgagcctcttaaagtcacccatgaggattgaaataaacttcttccaaacttctgttaatgttggtattttgacctcctcccataacagtgaatgatcgtgatgttatctagaatagcaaatcctttccagaagattttccatctccttttcccagattcatcagaggagtcattatgtacggcagctgtaagcttcagtagaattgaagacagttagggccctgctctggattaggctctggcttagggaatgttgtgggtggtttgatcttgtatccaaacttctaaaactttcttcacttttcctttgcattcacaacttggctaaccttagtgctagacacctagctttcagcctgtgctttcagcacctttctcattaaggtgaatcatttctagcttttgatttcaaatgagagacttgcaactcttcctttcacttgaacacttagaagccactgtaggtttattaagtggcctaatttcaatactgttgtatctcagacagtagagaggccctaggcatgatcctgattgagtaaagctgcactgaatcctcaaggatgtgaagatcaaaaagctttcaaatattctacctcaagtagatggtgatctctttaaagggtgaatgatgcattccgcttctccttttttcctgggtgccatggagggcatgttgatggtgggaggcagacagattcctgggcagaaaggggtggatccttggtgaaaccccacctttaatccagagacagcctgaggcctgggggtcagactgtcagttctgggtagtctgtagaccaaagtgagaacttatggagctttttccaggcccacccatggctgcccacagaccaatcagcatgcacttcctcccttctgaccccttaaaaaccccagactctgccagactcacacagacgtcaggattaccagctgtgggaaggagatacccactttgggtctcctcagctagtcaggacgacctgcctgcagaaagaaggtgcccaccgtggctctcctaagagttgttttgttgctcagtgaagctcctctctgccttgctcgctctccggttgtccatgtgcttcattcttcctcctgcgtacataacagccagcataatggatgaaatccatgctatttcactgtag

SEQ ID NO: 11061 - RNA, 6924 nt, Homo sapiens
  source 1..6924: mol_type = other RNA
ctgaatagctgggactacaggtgcacatcaccacatccaggtaattattttactttttgaatcatgatatgtagcaaccaatctgggaattatttattcataaaagataacattttcctgctaactccaacctcagaaaaaatgtattatgcctgactcaaatatgtcattatttttatgagaaaaagagtcatattgaagtaattatgtctatatgtaataattatcattatttgagataatttgcattggggagaaaagcaggcaatcagaaattacatattcaaggctgggcgcagtggctcacgcctgtaatcccagcactttgggaggcagaggcgagtgaatcacctgaggtcagagttcaagaccagcctgaccaacaaggagaaaccccatctctactaaaacaaaacaaaacaaaacaaaacaaaaaaagccacaaaattagccgggcatggtggcacatgcctgtaattccagttactcgggaggctgaggcaggagaattgcttgaacctgggaggcagaggttgtagtaagccgagattgtgccactgcacgccagcctgggcgacaagaacgagactcagtctcaaaaaaaaaaaaaaagaaagaaagaaagaaattacatattcaggttctagcaaatgcagttctctaataaacactaaataaatcataatacaagttacagttaaacctaattgttttactatataggatgtatcttttttgtacctatattttatcttcctttgcttctctggcctctattgggaggcagcacggtagtgaacacctcggggatctttctggttacgtaaacctgagttttaattttggttcatactaccttttaactttgggtagtctgctgagcttgttttttgttttcactcatctgtcatatcaagctagtaataattctgccatggttttggttttcatattgaaaggcattacataagcaaaatgcataacatataaatattagttccctttccactatgcatccaatctccctattaaattaagcctaaaaataataatttttgttttattaaaagccttccacattctacatatgaaagggattttttaaaggtgttttagataaaaaatgtttcaaccaactgaccaagaatatctcttcatatttatgtcatctacataaaaacttacatttatatcatatatcttttagtcttcttttctatattcttgattgtcatgttgtacagccagaaaagaatgagtataaattatctagattttttaaagtgcacattcaaacatagaaaatctaattattttacttgtttcttagtattaggctgaggccaatgagtccatgagctaaagggttgaaacttggcaccaaaaaagtgattgtttatgagtcctgtagatttatactgagaaaacatcatgtcttccaatgtgaaatacactaaaacctgattttttgtctcttaaggtgtgctaggtgaatgcaaaaaggatcaggaaagggggtgaggataggtcaggaaaagtgcaaacacaatgttctattcataaattagtgatggcatatttaaggttaagtagtaaaaaatatggggggctcagttaacacgaatgaaaaaatagttaaagtagccatgaattatctggataccttgatttaatgacaccctttcttctgtacaatttcataatgtgggaatagagattagtggggattgtagtggtataccctgactttgcttcatgatatctcaaatgtttaaaacctattattccctagagaaagaaatatgttcatactaattgttgcagaggcagaagccaaatatatctcctcctccatttatgtgactatatagtaatgaaaatcctaggttgatacacttttctcaatcttggaaagattctgctaaagcagcaaatcttctaacaagttcaagagggtggggagagtgaacaagtagaataatttatattaccctggaacaattctgaatcctgtaggtatttatgtcactgtttcaattgtgttctggtttaactgtcaatatttatgcatagcagttaacgtgtgtgcatatttgtaactgtgcagtgctactgccaggtgtgactgtacaaatcatgtgctttgaatgtgcaagttttactttcttttctaacaatttaatacagtgttagaaataaataacgaatgaagacaaccaaagagcagccagacaaatgtgaactggttttgacgtgacgagaaactcatcagtaagtaaataaacctcctccctggagaaggccactgaaatgcacccaggaggatgtctctactagaaggtaataaaaaatatatataatgtagtctttgacctaaaacctcatgattattactttgccatttatttccccctggtatctgatgttcatattagtttaatgtgccttttcagagaattcaagacactttttggaaagtagaatttttttttgaaaatttatgattggagaggtactacacaatttagaggttacatttcttgacaaatctgagttgaataaaaaagaactaaaaatataaacatagctaattcaagaatcaagatcgggtgaaactaaattaaaaacagccataaagtcccacattttccctaatttatttacctatgatattggcacatcttgttttacttaacatttgaaaaatacaaatatctcttcatatgcaaaagagcaaatgttaaatgaaaaactgaattttatatagcttcctaaatatgagccacatgcttaagcagtgaattaactttatgaatcaaatgtttaatgttaactattacaaaagcctggtatccaggtgcaatctcaccagaaaaaaatagcacctgcctttattacaataaaaaaaatggctaattccctttgacatcttaagagtgacactactttgtcaagcactaaatactttttaaattaatcatgttaaacttcagatttatagatataaatattgtatttataactttagtcataatgtacaatttctttcttgtttaaaagtactttctcactcaaaatggtatttatagtttaaaaagaatatgcctctgtattcaggagtgattcaaattcccagatgttttcacatagttatgaaaatgggaaagtgctgaattaaactgggctgcaatatttcaagttttttgctatcaggttataaactatacctacgattgcaagtcatacagtgcctctatttctagaaggcttttaaagtttcctggcttagttatgtccaaaggcagcaggaagtctcatcagtagagggcagaattttcaagtgctgccattcttatcccaggaggcatttccagtggttgagcacaaggcctgtttgtagtttgcttttgctcttgcattttgtggaagggaaggaactgagagagcttagagggttcattaaaaccacccctcactctcttagtcgtagtcagatggagtattcataacagtaacctccaattaccactatgtgttgggaaaaattagaattcggtctacttacaatcctgccaactaggattttactttgatatttcagtataacagtgaatctggattgatgcctgattaaaataaaatccctgattattactttctggattacgaactaaaatccctgtaaaatcaatggatgtgactcattgttaagagtcatgcagacttttacatattaggtaagaattctaaaaattatttgagggttctattctctagcaccaggtactaatgctccctactcaaaaaaaatcatgtgcatggattaatcaagtctaacagtgctcagatttaatggtttaacattgattttcttttctttgtcaaacttatatatgcaaatatttttatagtagtcagatgttatttttgaataaggatcaccctcatttttacccatgtgcttatctttaaaaccaacattgtaaagtagcacgcagacatatgtttcttttatcttcatggattatttttaccttaaaaataaattatcatttttttttttgaatttgggttttattctccagatactctgtgtacatgtgggtaagtatgtgggagtatgtgtgtttgtgtgtaagaggggataattaattgtctctcaactctatctcatactttaatatcaaataaaaaatgaaatgtataaagggtcactttgtaggattaggcatcctccttctacctacttaaaccaggggtttgggattcagaattctccatataaccaagaccgaaagtcactggaagactttaaaattagtattttaaccaccacacccagagtcaggtatggaaataaacctatagcatggattctttctatgcataatctcaaaatttaactacccaaataagtaagtttttaaaaactaatttaaaatttgccattgaggaaaatatcacctccatccttaattgtgactcctcatttcagctaaaaccttttctaatactttaaaaaaacaaaatgaaaaacaaactcctagataaagtcataaacactgaaatcagagatgtgattcttgttaaatgttagtttctctttctgaggttacactctgtgcatttgaaactttgacgttaacatcttccgaatgtttagatttgctcaagggttcagattctctggtcttctgccttgcattttcctccttcctttcctttgcaagcaatctatagttgatagcattgccaatgagcagccacacgcttgctgctaccacaatagccccacaggacatgtacatgtatttatattctccagttaaatccaccaatttacctgcaagaggagggccaagaagaactgggccacactccacaattgtgacaagtccgacggcactggaaaatcttggtgcacccacgaggtccatgagagtttcaaagagaacactgctaacactcccaaatccaaggccaaaaaatacagcatataataccaggcttgtgtagtcctgtgccagtgggcacaagaggtgacacactccattgaacatgattgcaaaactgaagaagtactgaattcgaggtcgaatatatttggagtttgcaattaatcctacagaaggcctagcaaacatatcaacgaaagccataacagatagcagaaaagctgccgagtactcatcaattccttggtctttagcatatggagccaagaatataatgggggcaaaaaaacctaggaacataatgacatttccagacagatatatcagaaatcctctatgcttaaaaagggagaaatctaaatacttattaactttttcccaagttgatttcttcgttttgattttctttgggcttgaatcatcttctgttttgccagtcttatttttagacttagaagtggtttgattgggtccaaggggtctcatgagggaaccagccacacaggcattcaaaagtagacttcccaaaatcaggaagcttcctttccagccaaaagtattaaaaaggtactgattgaaaggagccaatgaacttaagaaaacaggacttcctgccatggccaatccatttgccatgggtcgcttcctatagaagtatttgccaattatggttaaggcgggttgcaggttgaaggctaaacctaaacctgtaatgaatcccatagtgaggtacagctgtaccacgctgctactaaaggaggccaacaccattccaagacagcataataagcctcctgctatcaccaccggccggctgccgtatttattcaccaaaacactacttacaggacttcactgaagtcctgagcctcttaaagtcacccatgaggattgaaataaacttcttccaaacttctgttaatgttggtattttgacctcctcccataacagtgaatgatcgtgatgttatctagaatagcaaatcctttccagaagattttccatctccttttcccagattcatcagaggagtcattatgtacggcagctgtaagcttcagtagaattgaagacagttagggccctgctctggattaggctctggcttagggaatgttgtgggtggtttgatcttgtatccaaacttctaaaactttcttcacttttcctttgcattcacaacttggctaaccttagtgctagacacctagctttcagcctgtgctttcagcacctttctcattaaggtgaatcatttctagcttttgatttcaaatgagagacttgcaactcttcctttcacttgaacacttagaagccactgtaggtttattaagtggcctaatttcaatactgttgtatctcagacagtagagaggccctaggcatgatcctgattgagtaaagctgcactgaatcctcaaggatgtgaagatcaaaaagctttcaaatattctacctcctgcgtacataacagccagcataatggatgaaatccatgctatttcactgtaggtagtgtggaatatttgctgaatttctttgaagaatacggtgacagctttggggaatgcataggaaaatccaatggagataaaagctgctccaaccacaatccaaccccatcctccatctggaggtggatgcacaggtggggcacttggcattggtggcatttctgctcctctagtggaaattcaagtaacctggcgacaggtgtttagaaacatggtcttccatttcaccaagacataagtttccctgatctatggactcctctccccacctgaggcagaagtttccttgtgaaccattgctctttttagaatcctgaacatacttagttccatctatctctttgtcactcaacactttgtcagctagtctcaggattctatgaccccttcccctagctcacttgagtaatcataatatgggaaaactaatctaaatgccaactctgagaag

SEQ ID NO: 11062 - RNA, 6837 nt, Homo sapiens
  source 1..6837: mol_type = other RNA
ctgaatagctgggactacaggtgcacatcaccacatccaggtaattattttactttttgaatcatgatatgtagcaaccaatctgggaattatttattcataaaagataacattttcctgctaactccaacctcagaaaaaatgtattatgcctgactcaaatatgtcattatttttatgagaaaaagagtcatattgaagtaattatgtctatatgtaataattatcattatttgagataatttgcattggggagaaaagcaggcaatcagaaattacatattcaaggctgggcgcagtggctcacgcctgtaatcccagcactttgggaggcagaggcgagtgaatcacctgaggtcagagttcaagaccagcctgaccaacaaggagaaaccccatctctactaaaacaaaacaaaacaaaacaaaacaaaaaaagccacaaaattagccgggcatggtggcacatgcctgtaattccagttactcgggaggctgaggcaggagaattgcttgaacctgggaggcagaggttgtagtaagccgagattgtgccactgcacgccagcctgggcgacaagaacgagactcagtctcaaaaaaaaaaaaaaagaaagaaagaaagaaattacatattcaggttctagcaaatgcagttctctaataaacactaaataaatcataatacaagttacagttaaacctaattgttttactatataggatgtatcttttttgtacctatattttatcttcctttgcttctctggcctctattgggaggcagcacggtagtgaacacctcggggatctttctggttacgtaaacctgagttttaattttggttcatactaccttttaactttgggtagtctgctgagcttgttttttgttttcactcatctgtcatatcaagctagtaataattctgccatggttttggttttcatattgaaaggcattacataagcaaaatgcataacatataaatattagttccctttccactatgcatccaatctccctattaaattaagcctaaaaataataatttttgttttattaaaagccttccacattctacatatgaaagggattttttaaaggtgttttagataaaaaatgtttcaaccaactgaccaagaatatctcttcatatttatgtcatctacataaaaacttacatttatatcatatatcttttagtcttcttttctatattcttgattgtcatgttgtacagccagaaaagaatgagtataaattatctagattttttaaagtgcacattcaaacatagaaaatctaattattttacttgtttcttagtattaggctgaggccaatgagtccatgagctaaagggttgaaacttggcaccaaaaaagtgattgtttatgagtcctgtagatttatactgagaaaacatcatgtcttccaatgtgaaatacactaaaacctgattttttgtctcttaaggtgtgctaggtgaatgcaaaaaggatcaggaaagggggtgaggataggtcaggaaaagtgcaaacacaatgttctattcataaattagtgatggcatatttaaggttaagtagtaaaaaatatggggggctcagttaacacgaatgaaaaaatagttaaagtagccatgaattatctggataccttgatttaatgacaccctttcttctgtacaatttcataatgtgggaatagagattagtggggattgtagtggtataccctgactttgcttcatgatatctcaaatgtttaaaacctattattccctagagaaagaaatatgttcatactaattgttgcagaggcagaagccaaatatatctcctcctccatttatgtgactatatagtaatgaaaatcctaggttgatacacttttctcaatcttggaaagattctgctaaagcagcaaatcttctaacaagttcaagagggtggggagagtgaacaagtagaataatttatattaccctggaacaattctgaatcctgtaggtatttatgtcactgtttcaattgtgttctggtttaactgtcaatatttatgcatagcagttaacgtgtgtgcatatttgtaactgtgcagtgctactgccaggtgtgactgtacaaatcatgtgctttgaatgtgcaagttttactttcttttctaacaatttaatacagtgttagaaataaataacgaatgaagacaaccaaagagcagccagacaaatgtgaactggttttgacgtgacgagaaactcatcagtaagtaaataaacctcctccctggagaaggccactgaaatgcacccaggaggatgtctctactagaaggtaataaaaaatatatataatgtagtctttgacctaaaacctcatgattattactttgccatttatttccccctggtatctgatgttcatattagtttaatgtgccttttcagagaattcaagacactttttggaaagtagaatttttttttgaaaatttatgattggagaggtactacacaatttagaggttacatttcttgacaaatctgagttgaataaaaaagaactaaaaatataaacatagctaattcaagaatcaagatcgggtgaaactaaattaaaaacagccataaagtcccacattttccctaatttatttacctatgatattggcacatcttgttttacttaacatttgaaaaatacaaatatctcttcatatgcaaaagagcaaatgttaaatgaaaaactgaattttatatagcttcctaaatatgagccacatgcttaagcagtgaattaactttatgaatcaaatgtttaatgttaactattacaaaagcctggtatccaggtgcaatctcaccagaaaaaaatagcacctgcctttattacaataaaaaaaatggctaattccctttgacatcttaagagtgacactactttgtcaagcactaaatactttttaaattaatcatgttaaacttcagatttatagatataaatattgtatttataactttagtcataatgtacaatttctttcttgtttaaaagtactttctcactcaaaatggtatttatagtttaaaaagaatatgcctctgtattcaggagtgattcaaattcccagatgttttcacatagttatgaaaatgggaaagtgctgaattaaactgggctgcaatatttcaagttttttgctatcaggttataaactatacctacgattgcaagtcatacagtgcctctatttctagaaggcttttaaagtttcctggcttagttatgtccaaaggcagcaggaagtctcatcagtagagggcagaattttcaagtgctgccattcttatcccaggaggcatttccagtggttgagcacaaggcctgtttgtagtttgcttttgctcttgcattttgtggaagggaaggaactgagagagcttagagggttcattaaaaccacccctcactctcttagtcgtagtcagatggagtattcataacagtaacctccaattaccactatgtgttgggaaaaattagaattcggtctacttacaatcctgccaactaggattttactttgatatttcagtataacagtgaatctggattgatgcctgattaaaataaaatccctgattattactttctggattacgaactaaaatccctgtaaaatcaatggatgtgactcattgttaagagtcatgcagacttttacatattaggtaagaattctaaaaattatttgagggttctattctctagcaccaggtactaatgctccctactcaaaaaaaatcatgtgcatggattaatcaagtctaacagtgctcagatttaatggtttaacattgattttcttttctttgtcaaacttatatatgcaaatatttttatagtagtcagatgttatttttgaataaggatcaccctcatttttacccatgtgcttatctttaaaaccaacattgtaaagtagcacgcagacatatgtttcttttatcttcatggattatttttaccttaaaaataaattatcatttttttttttgaatttgggttttattctccagatactctgtgtacatgtgggtaagtatgtgggagtatgtgtgtttgtgtgtaagaggggataattaattgtctctcaactctatctcatactttaatatcaaataaaaaatgaaatgtataaagggtcactttgtaggattaggcatcctccttctacctacttaaaccaggggtttgggattcagaattctccatataaccaagaccgaaagtcactggaagactttaaaattagtattttaaccaccacacccagagtcaggtatggaaataaacctatagcatggattctttctatgcataatctcaaaatttaactacccaaataagtaagtttttaaaaactaatttaaaatttgccattgaggaaaatatcacctccatccttaattgtgactcctcatttcagctaaaaccttttctaatactttaaaaaaacaaaatgaaaaacaaactcctagataaagtcataaacactgaaatcagagatgtgattcttgttaaatgttagtttctctttctgaggttacactctgtgcatttgaaactttgacgttaacatcttccgaatgtttagatttgctcaagggttcagattctctggtcttctgccttgcattttcctccttcctttcctttgcaagcaatctatagttgatagcattgccaatgagcagccacacgcttgctgctaccacaatagccccacaggacatgtacatgtatttatattctccagttaaatccaccaatttacctgcaagaggagggccaagaagaactgggccacactccacaattgtgacaagtccgacggcactggaaaatcttggtgcacccacgaggtccatgagagtttcaaagagaacactgctaacactcccaaatccaaggccaaaaaatacagcatataataccaggcttgtgtagtcctgtgccagtgggcacaagaggtgacacactccattgaacatgattgcaaaactgaagaagtactgaattcgaggtcgaatatatttggagtttgcaattaatcctacagaaggcctagcaaacatatcaacgaaagccataacagatagcagaaaagctgccgagtactcatcaattccttggtctttagcatatggagccaagaatataatgggggcaaaaaaacctaggaacataatgacatttccagacagatatatcagaaatcctctatgcttaaaaagggagaaatctaaatacttattaactttttcccaagttgatttcttcgttttgattttctttgggcttgaatcatcttctgttttgccagtcttatttttagacttagaagtggtttgattgggtccaaggggtctcatgagggaaccagccacacaggcattcaaaagtagacttcccaaaatcaggaagcttcctttccagccaaaagtattaaaaaggtactgattgaaaggagccaatgaacttaagaaaacaggacttcctgccatggccaatccatttgccatgggtcgcttcctatagaagtatttgccaattatggttaaggcgggttgcaggttgaaggctaaacctaaacctgtaatgaatcccatagtgaggtacagctgtaccacgctgctactaaaggaggccaacaccattccaagacagcataataagcctcctgctatcaccaccggccggctgccgtatttattcaccaaaacactacttacaggacttcactgaagtcctgagcctcttaaagtcacccatgaggattgaaataaacttcttccaaacttctgttaatgttggtattttgacctcctcccataacagtgaatgatcgtgatgttatctagaatagcaaatcctttccagaagattttccatctccttttcccagattcatcagaggagtcattatgtacggcagcttcagtagaattgaagacagttagggccctgctctggattaggctctggcttagggaatgttgtgggtggtttgatcttgtatccaaacttctaaaactttcttcacttttcctttgcattcacaacttggctaaccttagtgctagacacctagctttcagcctgtgctttcagcacctttctcattaaggtgaatcatttctagcttttgatttcaaatgagagacttgcaactcttcctttcacttgaacacttagaagccactgtaggtttattaagtggcctaatttcaatactgttgtatctcagacagtagagaggccctaggcatgatcctgattgagtaaagctgcactgaatcctcaaggatgtgaagatcaaaaagctttcaaatattctacctcaagtagatggtgatctctttaaagggtgaatgatgcattccgcttctccttttttcctcctgcgtacataacagccagcataatggatgaaatccatgctatttcactgtaggtagtgtggaatatttgctgaatttctttgaagaatacggtgacagctttggggaatgcataggaaaatccaatggagataaaagctgctccaaccacaatccaaccccatcctccatctggaggtggatgcacaggtggggcacttggcattggtggcatttctgctcctctagtggaaattcaagtaacctggcgacaggtgtttagaaacatggtcttccatttcaccaagacataagtttccctgatctatggactcctctccccacctgaggcagaagtttccttgtgaaccattgctctttttagaat

SEQ ID NO: 11063 - RNA, 5361 nt, Homo sapiens
  source 1..5361: mol_type = other RNA
ctgaatagctgggactacaggtgcacatcaccatgcccgactaatttttgtatttttagtagaaactgggtatcaccatgttgtccaggctggtctcgaactcctggcctcaagtgatctgcctgtcttagcctcccaaagttctgggattacaggcgtgagccactgcacctggccagttctagtagttattaaaccatgcattggaagaccctgctggaatataagatgcagagcacagaaagaaaactaagtgaagaaagaattgtttcggagccttgtaaggaatactcacgtcctccttctccaagctgggctccctgaagttggcaatttcatcaaaacagtatccacttaaaagtacccttaactttttcttccaaagttacacagtagccccaagttctacaatgcccacttcatgttttcctgaggcaccctggagacgccaaaagcatttgagaatgaacgggcctttttttttttttttttttcttttttgagcccaggctggagtgcagtggtgtgatctcggctcactgcaagctccgcctcctgggttcacaccattcccctgcctcagcctccggagtagctgggactacaggcacccgccaccaagcccggctaatttttttgtatttttagtagagaaggggtttcaccgtattagccaggatggtgaacatgcctttaatgcagccttgaacaggaattggccaagccttgccaacttgataaggagcaaaaaaggctctaaaggtgtatggctccccagatttctggagggcatccaaatgaatgagaacagggctgcaggtagtcacctgcagcatcctcctgggcacgatgacagagggaagtgtctctaccaagatccatcatgggggacaggttcccatagccccggacacacaacctaaaaaccgtggttctgtggaccgacacccgtaagaccctagagctggaaaggcccacctgtgaaggtcattcagcactccaccacccaccccctaccagtacagctgaaagctctggaccagcgggtgacaggctgatgcatctgacatttgggcggagaccttcccatgacagcaggatgcctcaggtgctgggaccactgctgcctccctcctttctcagcagtcgtctatgttcctctgagactgctggctgagaagccatcaggtgggttccctgatgagactgacaccctctctgctctgctgggagccttccaacactgcagccacctacagtcacatgcatgcctgccacctccccagtggcctctgcatggaatctcccagagaaattccacgttccaggaaggttgtgcatccattaattttcattgttattcatggggaaacccagtgccaggcttcttgtggaccatgcagatggtttttcagcccagcccacagccctgccctgtgggtagtgggattccccggaggctggtgaggacagctgcagcagagtcctaagcagacatatgggagaggtcagagaactggcgagcctgggcctctgaagcagagaagcagaggacattcaggaggtgcagtgtctggtgctacagaggctgaagaaggccagagttgacaattgggataagcagctttcagctacgtggggcatggtgggtggtgcaaaggaaggggtacagacagcccagataagaagctgcctgggaaagaaagggagggagccatagggcctcggcaagtttttaggatgggaaaggaaggccagcgataggaagacgggacaggaaaaataacgttgacaagatcctgagagggggtggaccagggttgaggagggggtacaggaaagaccccaaggctttaaagttagcatgtgcatggtgaggtgagaagagggtgcaaatgccacagctggcctccaaccagggaaggcggggattcaggacaggccagtgctaggtggggagtgcacaggaggcctgccctgtgcctctgtgcggacagccgatgctgggcggagactgccacgtgaccggctctcatccttgctttctttccattcctcatccaactattcagagtcacatgatatggctgagaacagccagaagggtctatagttgaaagataaacccaactctgcaaaaatcgcaccgagacttcatcctaaaccaggtctacaggaatagatgggtcaggcctgcaggagccttccaggagctctggcagggagggtctgtggccacccactcccccaggggaggctgggtcagaggcatctagtgaggtgggcactgccaccaacccccttcacagaaaggccggcacacccaggacacacagctcatgcagcagcagtgcccaggcttcaatcccatgtccccacttcgactcagtgtccccaagctcttctgcttggatcaataaatagtatcgcacaggggtggacagaaataacctaaaacaatgtttcctctagacctatggagttgaagtttctccagctctcacttatagcgggggataaaccacaagccaacttgtgcggctgtggccggcacacaagggcaactgaaagtgctgccatacagaatcttaaaaaaaaaaaaaattactcaatgaaatgtaagtcagattgtgctgatgatggactgcctttaccatccatccttctgtaaggtctacataccctatcccttggttcctctggcagccgcgtttaccactgagatgcttagcaatatctcaatagtgaccccaaacaaaaatgaccaaaacagcattaatataaagatatattccataaaagagtttggcagtcaaagagaagcatcacacttccgaaaaacacaagcattcttctcctagtctacagagaattgtgtaaaaaaaaaaaaatcatcatcaacagccaccagtatacaccacactagaatgtacactccggcaagtaaattaaggttgcagtccatccctgaacgatgagaagtggtctgagctatggcaaagtgttagaaagtagcccagctagacaaatgccccagctatccccaggggagttattcagtacttaagacttcatttccaagagcagccccagaaaagccctgacaggaagggtggaccagtgatcaccgatatcccattaggggcggtcaccagaaacaaaatgcctggagcttctgagcagctgcagcctggggttgtggctaggcacggggtgtggttgcagaagaacggctgtctccggggagaggcaaatggcaggccagccagccctgggtacatggccacaagaggagccctggccaacagtttcaggctggccatcttgggctggggctccctgggcttgcagtggggagggtcaggattcaaattctgggtgacaatttcagtagcaccaagaccagaagacagtgaggccacgctggggagtgggggagtgcttgtatgtgggatgcatggagggaggctgcagtatgtggaggagaaagagaggctgttgtgggctggttcttaagacactcaaggggactcaaagggtcggctccagccatggacactatctaaggctgctcagaggagaatgctggaggagaggaagaggaagtgaaatggtgtgagaacattcttacccctataaataaactatttacacactttaagaaaaggagagccggctctcagtgaagaaccatgcccaccgcgccaccggcgccatcagggcttaatgctatcaagaccagaggcagttccggcgccaggagaatagctggtggacacagggggacagtggacaaggcactcccgtggcaccagtccacgcactggctcaggcttacttcacttgaacatggctgaggatcctgcaaacaacccctgatatgtgcatgtcccagcagactgcgctggcactcagaggcccagcggggccacgtccgcctcccgttacgggcaggcccccatgctgctttgcttgatggagagagatgccctgtccacgcctgtgggtccctctacccacggcccacccacagatgtggatgacccaaagcagatgtctggatgccagtggagaggggaccagggtgtcctgcagacatgcttgagctgcagggggtctgagtcaagccctcctggcagccacaggagccctctctgtctttcagagtcaccactcccacataaagacacattctctgtctctgggtagactccagagggatgcagtcacaagtttgggcaggtaacaagggggacccttggtcttcagcaccagcaagcagaaacagagaggtcacgtcacgctgatgcttaagatggggcactggctctgggggtgtcggctcctctccctctggacgtagggctgatggcagagaaaggctctggcctcccagcgtggctcagctcggctccctcaactctgctcctcagaagtgatggccggccttcactgcctcgatgtctgagatcagcgtccttgccaggaagatgccaaatatctgcaacagcgagatggcgatgaagacgccagccacaatgtaaatgttccgcgggagccagctttccagcgcctggatgcagcctttcgtgaagatggactcatcccacttgctcttcagctgaatcctgacatcatatccacactgtgtgttcacaactttttgcgcaggatctggcacgcagcaggagaaggggaccccgcacttctctcggctgtagctggcaccgctgcaattgaagtagacgttgaggtcccagtcttcagggccatatgcgccacagcactggttagctttctgaagggagtcgatgaggttttgcagatcgatatcgtcccggtaggacttgatgttgctctcgaagaactcccggaaccggtccctcacccagtcctggaacaggaaggccagcacggccacagccagctccaggaagaagatgagcacgatggtgccacagaaaaagttgagcaagcagatattctcccgcagagcccccacgcagccggcgaaccccagggtgaacatcaccacgcccaccatcaggaccagcaccacagggtcgattccatgcatccgggtcactttggtgaggtcggacagcacacccttttcgctccatgcccacagcccgactccaaggaagacaactccagccaaccagaagatgatgttgtagctgaaaaggaggtacttgtaccagcagctgaccttggcgttagagtatctataatagtgcatcttctgagaagcagaatcaactcacagggctccctgctttcgactccaccccaagtcccgcgcgcggcggcggcagcggcggcgcggcccggctcggccgaggaagttagagcaagttc

SEQ ID NO: 11064 - RNA, 5321 nt, Homo sapiens
  source 1..5321: mol_type = other RNA
ctgaatagctgggactacaggtgcacatcaccatgcccgactaatttttgtatttttagtagaaactgggtatcaccatgttgtccaggctggtctcgaactcctggcctcaagtgatctgcctgtcttagcctcccaaagttctgggattacaggcgtgagccactgcacctggccagttctagtagttattaaaccatgcattggaagaccctgctggaatataagatgcagagcacagaaagaaaactaagtgaagaaagaattgtttcggagccttgtaaggaatactcacgtcctccttctccaagctgggctccctgaagttggcaatttcatcaaaacagtatccacttaaaagtacccttaactttttcttccaaagttacacagtagccccaagttctacaatgcccacttcatgttttcctgaggcaccctggagacgccaaaagcatttgagaatgaacgggcctttttttttttttttttttcttttttgagcccaggctggagtgcagtggtgtgatctcggctcactgcaagctccgcctcctgggttcacaccattcccctgcctcagcctccggagtagctgggactacaggcacccgccaccaagcccggctaatttttttgtatttttagtagagaaggggtttcaccgtattagccaggatggtgaacatgcctttaatgcagccttgaacaggaattggccaagccttgccaacttgataaggagcaaaaaaggctctaaaggtgtatggctccccagatttctggagggcatccaaatgaatgagaacagggctgcaggtagtcacctgcagcatcctcctgggcacgatgacagagggaagtgtctctaccaagatccatcatgggggacaggttcccatagccccggacacacaacctaaaaaccgtggttctgtggaccgacacccgtaagaccctagagctggaaaggcccacctgtgaaggtcattcagcactccaccacccaccccctaccagtacagctgaaagctctggaccagcgggtgacaggctgatgcatctgacatttgggcggagaccttcccatgacagcaggatgcctcaggtgctgggaccactgctgcctccctcctttctcagcagtcgtctatgttcctctgagactgctggctgagaagccatcaggtgggttccctgatgagactgacaccctctctgctctgctgggagccttccaacactgcagccacctacagtcacatgcatgcctgccacctccccagtggcctctgcatggaatctcccagagaaattccacgttccaggaaggttgtgcatccattaattttcattgttattcatggggaaacccagtgccaggcttcttgtggaccatgcagatggtttttcagcccagcccacagccctgccctgtgggtagtgggattccccggaggctggtgaggacagctgcagcagagtcctaagcagacatatgggagaggtcagagaactggcgagcctgggcctctgaagcagagaagcagaggacattcaggaggtgcagtgtctggtgctacagaggctgaagaaggccagagttgacaattgggataagcagctttcagctacgtggggcatggtgggtggtgcaaaggaaggggtacagacagcccagataagaagctgcctgggaaagaaagggagggagccatagggcctcggcaagtttttaggatgggaaaggaaggccagcgataggaagacgggacaggaaaaataacgttgacaagatcctgagagggggtggaccagggttgaggagggggtacaggaaagaccccaaggctttaaagttagcatgtgcatggtgaggtgagaagagggtgcaaatgccacagctggcctccaaccagggaaggcggggattcaggacaggccagtgctaggtggggagtgcacaggaggcctgccctgtgcctctgtgcggacagccgatgctgggcggagactgccacgtgaccggctctcatccttgctttctttccattcctcatccaactattcagagtcacatgatatggctgagaacagccagaagggtctatagttgaaagataaacccaactctgcaaaaatcgcaccgagacttcatcctaaaccaggtctacaggaatagatgggtcaggcctgcaggagccttccaggagctctggcagggagggtctgtggccacccactcccccaggggaggctgggtcagaggcatctagtgaggtgggcactgccaccaacccccttcacagaaaggccggcacacccaggacacacagctcatgcagcagcagtgcccaggcttcaatcccatgtccccacttcgactcagtgtccccaagctcttctgcttggatcaataaatagtatcgcacaggggtggacagaaataacctaaaacaatgtttcctctagacctatggagttgaagtttctccagctctcacttatagcgggggataaaccacaagccaacttgtgcggctgtggccggcacacaagggcaactgaaagtgctgccatacagaatcttaaaaaaaaaaaaaattactcaatgaaatgtaagtcagattgtgctgatgatggactgcctttaccatccatccttctgtaaggtctacataccctatcccttggttcctctggcagccgcgtttaccactgagatgcttagcaatatctcaatagtgaccccaaacaaaaatgaccaaaacagcattaatataaagatatattccataaaagagtttggcagtcaaagagaagcatcacacttccgaaaaacacaagcattcttctcctagtctacagagaattgtgtaaaaaaaaaaaaatcatcatcaacagccaccagtatacaccacactagaatgtacactccggcaagtaaattaaggttgcagtccatccctgaacgatgagaagtggtctgagctatggcaaagtgttagaaagtagcccagctagacaaatgccccagctatccccaggggagttattcagtacttaagacttcatttccaagagcagccccagaaaagccctgacaggaagggtggaccagtgatcaccgatatcccattaggggcggtcaccagaaacaaaatgcctggagcttctgagcagctgcagcctggggttgtggctaggcacggggtgtggttgcagaagaacggctgtctccggggagaggcaaatggcaggccagccagccctgggtacatggccacaagaggagccctggccaacagtttcaggctggccatcttgggctggggctccctgggcttgcagtggggagggtcaggattcaaattctgggtgacaatttcagtagcaccaagaccagaagacagtgaggccacgctggggagtgggggagtgcttgtatgtgggatgcatggagggaggctgcagtatgtggaggagaaagagaggctgttgtgggctggttcttaagacactcaaggggactcaaagggtcggctccagccatggacactatctaaggctgctcagaggagaatgctggaggagaggaagaggaagtgaaatggtgtgagaacattcttacccctataaataaactatttacacactttaagaaaaggagagccggctctcagtgaagaaccatgcccaccgcgccaccggcgccatcagggcttaatgctatcaagaccagaggcagttccggcgccaggagaatagctggtggacacagggggacagtggacaaggcactcccgtggcaccagtccacgcactggctcaggcttacttcacttgaacatggctgaggatcctgcaaacaacccctgatatgtgcatgtcccagcagactgcgctggcactcagaggcccagcggggccacgtccgcctcccgttacgggcaggcccccatgctgctttgcttgatggagagagatgccctgtccacgcctgtgggtccctctacccacggcccacccacagatgtggatgacccaaagcagatgtctggatgccagtggagaggggaccagggtgtcctgcagacatgcttgagctgcagggggtctgagtcaagccctcctggcagccacaggagccctctctgtctttcagagtcaccactcccacataaagacacattctctgtctctgggtagactccagagggatgcagtcacaagtttgggcaggtaacaagggggacccttggtcttcagcaccagcaagcagaaacagagaggtcacgtcacgctgatgcttaagatggggcactggctctgggggtgtcggctcctctccctctggacgtagggctgatggcagagaaaggctctggcctcccagcgtggctcagctcggctccctcaactctgctcctcagaagtgatggccggccttcactgcctcgatgtctgagatcagcgtccttgccaggaagatgccaaatatctgcaacagcgagatggcgatgaagacgccagccacaatgtaaatgttccgcgggagccagctttccagcgcctggatgcagcctttcgtgaagatggactcatcccacttgctcttcagctgaatcctgacatcatatccacactgtgtgttcacaactttttgcgcaggatctggcacgcagcaggagaaggggaccccgcacttctctcggctgtagctggcaccgctgcaattgaagtagacgttgaggtcccagtcttcagggccatatgcgccacagcactggttagctttctgaagggagtcgatgaggttttgcagatcgatatcgtcccggtaggacttgatgttgctctcgaagaactcccggaaccggtccctcacccagtcctggaacaggaaggccagcacggccacagccagctccaggaagaagatgagcacgatggtgccacagaaaaagttgagcaagcagatattctcccgcagagcccccacgcagccggcgaaccccagggtgaacatcaccacgcccaccatcaggaccagcaccacagggtcgattccatgcatccgggtcactttggtgaggtcggacagcacacccttttcgctccatgcccacagcccgactccaaggaagacaactccagccaaccagaagatgatgttgtagctgaaaaggaggtacttgtaccagcagctgaccttggcgttagagtatctataatagtgcatcttctgagaagcagaatccgcgcgcggcggcggcagcggcggcgcggcccggctcggccgaggaagttagagcaagttc

SEQ ID NO: 11065 - RNA, 5482 nt, Homo sapiens
  source 1..5482: mol_type = other RNA
ctgaatagctgggactacaggtgcacatcaccatgcccgactaatttttgtatttttagtagaaactgggtatcaccatgttgtccaggctggtctcgaactcctggcctcaagtgatctgcctgtcttagcctcccaaagttctgggattacaggcgtgagccactgcacctggccagttctagtagttattaaaccatgcattggaagaccctgctggaatataagatgcagagcacagaaagaaaactaagtgaagaaagaattgtttcggagccttgtaaggaatactcacgtcctccttctccaagctgggctccctgaagttggcaatttcatcaaaacagtatccacttaaaagtacccttaactttttcttccaaagttacacagtagccccaagttctacaatgcccacttcatgttttcctgaggcaccctggagacgccaaaagcatttgagaatgaacgggcctttttttttttttttttttcttttttgagcccaggctggagtgcagtggtgtgatctcggctcactgcaagctccgcctcctgggttcacaccattcccctgcctcagcctccggagtagctgggactacaggcacccgccaccaagcccggctaatttttttgtatttttagtagagaaggggtttcaccgtattagccaggatggtgaacatgcctttaatgcagccttgaacaggaattggccaagccttgccaacttgataaggagcaaaaaaggctctaaaggtgtatggctccccagatttctggagggcatccaaatgaatgagaacagggctgcaggtagtcacctgcagcatcctcctgggcacgatgacagagggaagtgtctctaccaagatccatcatgggggacaggttcccatagccccggacacacaacctaaaaaccgtggttctgtggaccgacacccgtaagaccctagagctggaaaggcccacctgtgaaggtcattcagcactccaccacccaccccctaccagtacagctgaaagctctggaccagcgggtgacaggctgatgcatctgacatttgggcggagaccttcccatgacagcaggatgcctcaggtgctgggaccactgctgcctccctcctttctcagcagtcgtctatgttcctctgagactgctggctgagaagccatcaggtgggttccctgatgagactgacaccctctctgctctgctgggagccttccaacactgcagccacctacagtcacatgcatgcctgccacctccccagtggcctctgcatggaatctcccagagaaattccacgttccaggaaggttgtgcatccattaattttcattgttattcatggggaaacccagtgccaggcttcttgtggaccatgcagatggtttttcagcccagcccacagccctgccctgtgggtagtgggattccccggaggctggtgaggacagctgcagcagagtcctaagcagacatatgggagaggtcagagaactggcgagcctgggcctctgaagcagagaagcagaggacattcaggaggtgcagtgtctggtgctacagaggctgaagaaggccagagttgacaattgggataagcagctttcagctacgtggggcatggtgggtggtgcaaaggaaggggtacagacagcccagataagaagctgcctgggaaagaaagggagggagccatagggcctcggcaagtttttaggatgggaaaggaaggccagcgataggaagacgggacaggaaaaataacgttgacaagatcctgagagggggtggaccagggttgaggagggggtacaggaaagaccccaaggctttaaagttagcatgtgcatggtgaggtgagaagagggtgcaaatgccacagctggcctccaaccagggaaggcggggattcaggacaggccagtgctaggtggggagtgcacaggaggcctgccctgtgcctctgtgcggacagccgatgctgggcggagactgccacgtgaccggctctcatccttgctttctttccattcctcatccaactattcagagtcacatgatatggctgagaacagccagaagggtctatagttgaaagataaacccaactctgcaaaaatcgcaccgagacttcatcctaaaccaggtctacaggaatagatgggtcaggcctgcaggagccttccaggagctctggcagggagggtctgtggccacccactcccccaggggaggctgggtcagaggcatctagtgaggtgggcactgccaccaacccccttcacagaaaggccggcacacccaggacacacagctcatgcagcagcagtgcccaggcttcaatcccatgtccccacttcgactcagtgtccccaagctcttctgcttggatcaataaatagtatcgcacaggggtggacagaaataacctaaaacaatgtttcctctagacctatggagttgaagtttctccagctctcacttatagcgggggataaaccacaagccaacttgtgcggctgtggccggcacacaagggcaactgaaagtgctgccatacagaatcttaaaaaaaaaaaaaattactcaatgaaatgtaagtcagattgtgctgatgatggactgcctttaccatccatccttctgtaaggtctacataccctatcccttggttcctctggcagccgcgtttaccactgagatgcttagcaatatctcaatagtgaccccaaacaaaaatgaccaaaacagcattaatataaagatatattccataaaagagtttggcagtcaaagagaagcatcacacttccgaaaaacacaagcattcttctcctagtctacagagaattgtgtaaaaaaaaaaaaatcatcatcaacagccaccagtatacaccacactagaatgtacactccggcaagtaaattaaggttgcagtccatccctgaacgatgagaagtggtctgagctatggcaaagtgttagaaagtagcccagctagacaaatgccccagctatccccaggggagttattcagtacttaagacttcatttccaagagcagccccagaaaagccctgacaggaagggtggaccagtgatcaccgatatcccattaggggcggtcaccagaaacaaaatgcctggagcttctgagcagctgcagcctggggttgtggctaggcacggggtgtggttgcagaagaacggctgtctccggggagaggcaaatggcaggccagccagccctgggtacatggccacaagaggagccctggccaacagtttcaggctggccatcttgggctggggctccctgggcttgcagtggggagggtcaggattcaaattctgggtgacaatttcagtagcaccaagaccagaagacagtgaggccacgctggggagtgggggagtgcttgtatgtgggatgcatggagggaggctgcagtatgtggaggagaaagagaggctgttgtgggctggttcttaagacactcaaggggactcaaagggtcggctccagccatggacactatctaaggctgctcagaggagaatgctggaggagaggaagaggaagtgaaatggtgtgagaacattcttacccctataaataaactatttacacactttaagaaaaggagagccggctctcagtgaagaaccatgcccaccgcgccaccggcgccatcagggcttaatgctatcaagaccagaggcagttccggcgccaggagaatagctggtggacacagggggacagtggacaaggcactcccgtggcaccagtccacgcactggctcaggcttacttcacttgaacatggctgaggatcctgcaaacaacccctgatatgtgcatgtcccagcagactgcgctggcactcagaggcccagcggggccacgtccgcctcccgttacgggcaggcccccatgctgctttgcttgatggagagagatgccctgtccacgcctgtgggtccctctacccacggcccacccacagatgtggatgacccaaagcagatgtctggatgccagtggagaggggaccagggtgtcctgcagacatgcttgagctgcagggggtctgagtcaagccctcctggcagccacaggagccctctctgtctttcagagtcaccactcccacataaagacacattctctgtctctgggtagactccagagggatgcagtcacaagtttgggcaggtaacaagggggacccttggtcttcagcaccagcaagcagaaacagagaggtcacgtcacgctgatgcttaagatggggcactggctctgggggtgtcggctcctctccctctggacgtagggctgatggcagagaaaggctctggcctcccagcgtggctcagctcggctccctcaactctgctcctcagaagtgatggccggccttcactgcctcgatgtctgagatcagcgtccttgccaggaagatgccaaatatctgcaacagcgagatggcgatgaagacgccagccacaatgtaaatgttccgcgggagccagctttccagcgcctggatgcagcctttcgtgaagatggactcatcccacttgctcttcagctgaatcctgacatcatatccacactgtgtgttcacaactttttgcgcaggatctggcacgcagcaggagaaggggaccccgcacttctctcggctgtagctggcaccgctgcaattgaagtagacgttgaggtcccagtcttcagggccatatgcgccacagcactggttagctttctgaagggagtcgatgaggttttgcagatcgatatcgtcccggtaggacttgatgttgctctcgaagaactcccggaaccggtccctcacccagtcctggaacaggaaggccagcacggccacagccagctccaggaagaagatgagcacgatggtgccacagaaaaagttgagcaagcagatattctcccgcagagcccccacgcagccggcgaaccccagggtgaacatcaccacgcccaccatcaggaccagcaccacagggtcgattccatgcatccgggtcactttggtgaggtcggacagcacacccttttcgctccatgcccacagcccgactccaaggaagacaactccagccaaccagaagatgatgttgtagctgaaaaggaggtacttgtaccagcagctgaccttggcgttagagtatctataatagtgcatcttctgagaagcagaatctcttaccagaatcccagaagccactttagagacaactgccccagctctcaggctcccagctcaggccagcacagcctaaggagggaggagccagttcctccagctatctagctgaaaggcacaggctctaggccttctccctggctgctcagttgggaggcagtacagaccgcaaggggtgaagagtttcaaccccagcctgcccaggcccacttaagctct

SEQ ID NO: 11066 - RNA, 5502 nt, Homo sapiens
  source 1..5502: mol_type = other RNA
ctgaatagctgggactacaggtgcacatcaccatgcccgactaatttttgtatttttagtagaaactgggtatcaccatgttgtccaggctggtctcgaactcctggcctcaagtgatctgcctgtcttagcctcccaaagttctgggattacaggcgtgagccactgcacctggccagttctagtagttattaaaccatgcattggaagaccctgctggaatataagatgcagagcacagaaagaaaactaagtgaagaaagaattgtttcggagccttgtaaggaatactcacgtcctccttctccaagctgggctccctgaagttggcaatttcatcaaaacagtatccacttaaaagtacccttaactttttcttccaaagttacacagtagccccaagttctacaatgcccacttcatgttttcctgaggcaccctggagacgccaaaagcatttgagaatgaacgggcctttttttttttttttttttcttttttgagcccaggctggagtgcagtggtgtgatctcggctcactgcaagctccgcctcctgggttcacaccattcccctgcctcagcctccggagtagctgggactacaggcacccgccaccaagcccggctaatttttttgtatttttagtagagaaggggtttcaccgtattagccaggatggtgaacatgcctttaatgcagccttgaacaggaattggccaagccttgccaacttgataaggagcaaaaaaggctctaaaggtgtatggctccccagatttctggagggcatccaaatgaatgagaacagggctgcaggtagtcacctgcagcatcctcctgggcacgatgacagagggaagtgtctctaccaagatccatcatgggggacaggttcccatagccccggacacacaacctaaaaaccgtggttctgtggaccgacacccgtaagaccctagagctggaaaggcccacctgtgaaggtcattcagcactccaccacccaccccctaccagtacagctgaaagctctggaccagcgggtgacaggctgatgcatctgacatttgggcggagaccttcccatgacagcaggatgcctcaggtgctgggaccactgctgcctccctcctttctcagcagtcgtctatgttcctctgagactgctggctgagaagccatcaggtgggttccctgatgagactgacaccctctctgctctgctgggagccttccaacactgcagccacctacagtcacatgcatgcctgccacctccccagtggcctctgcatggaatctcccagagaaattccacgttccaggaaggttgtgcatccattaattttcattgttattcatggggaaacccagtgccaggcttcttgtggaccatgcagatggtttttcagcccagcccacagccctgccctgtgggtagtgggattccccggaggctggtgaggacagctgcagcagagtcctaagcagacatatgggagaggtcagagaactggcgagcctgggcctctgaagcagagaagcagaggacattcaggaggtgcagtgtctggtgctacagaggctgaagaaggccagagttgacaattgggataagcagctttcagctacgtggggcatggtgggtggtgcaaaggaaggggtacagacagcccagataagaagctgcctgggaaagaaagggagggagccatagggcctcggcaagtttttaggatgggaaaggaaggccagcgataggaagacgggacaggaaaaataacgttgacaagatcctgagagggggtggaccagggttgaggagggggtacaggaaagaccccaaggctttaaagttagcatgtgcatggtgaggtgagaagagggtgcaaatgccacagctggcctccaaccagggaaggcggggattcaggacaggccagtgctaggtggggagtgcacaggaggcctgccctgtgcctctgtgcggacagccgatgctgggcggagactgccacgtgaccggctctcatccttgctttctttccattcctcatccaactattcagagtcacatgatatggctgagaacagccagaagggtctatagttgaaagataaacccaactctgcaaaaatcgcaccgagacttcatcctaaaccaggtctacaggaatagatgggtcaggcctgcaggagccttccaggagctctggcagggagggtctgtggccacccactcccccaggggaggctgggtcagaggcatctagtgaggtgggcactgccaccaacccccttcacagaaaggccggcacacccaggacacacagctcatgcagcagcagtgcccaggcttcaatcccatgtccccacttcgactcagtgtccccaagctcttctgcttggatcaataaatagtatcgcacaggggtggacagaaataacctaaaacaatgtttcctctagacctatggagttgaagtttctccagctctcacttatagcgggggataaaccacaagccaacttgtgcggctgtggccggcacacaagggcaactgaaagtgctgccatacagaatcttaaaaaaaaaaaaaattactcaatgaaatgtaagtcagattgtgctgatgatggactgcctttaccatccatccttctgtaaggtctacataccctatcccttggttcctctggcagccgcgtttaccactgagatgcttagcaatatctcaatagtgaccccaaacaaaaatgaccaaaacagcattaatataaagatatattccataaaagagtttggcagtcaaagagaagcatcacacttccgaaaaacacaagcattcttctcctagtctacagagaattgtgtaaaaaaaaaaaaatcatcatcaacagccaccagtatacaccacactagaatgtacactccggcaagtaaattaaggttgcagtccatccctgaacgatgagaagtggtctgagctatggcaaagtgttagaaagtagcccagctagacaaatgccccagctatccccaggggagttattcagtacttaagacttcatttccaagagcagccccagaaaagccctgacaggaagggtggaccagtgatcaccgatatcccattaggggcggtcaccagaaacaaaatgcctggagcttctgagcagctgcagcctggggttgtggctaggcacggggtgtggttgcagaagaacggctgtctccggggagaggcaaatggcaggccagccagccctgggtacatggccacaagaggagccctggccaacagtttcaggctggccatcttgggctggggctccctgggcttgcagtggggagggtcaggattcaaattctgggtgacaatttcagtagcaccaagaccagaagacagtgaggccacgctggggagtgggggagtgcttgtatgtgggatgcatggagggaggctgcagtatgtggaggagaaagagaggctgttgtgggctggttcttaagacactcaaggggactcaaagggtcggctccagccatggacactatctaaggctgctcagaggagaatgctggaggagaggaagaggaagtgaaatggtgtgagaacattcttacccctataaataaactatttacacactttaagaaaaggagagccggctctcagtgaagaaccatgcccaccgcgccaccggcgccatcagggcttaatgctatcaagaccagaggcagttccggcgccaggagaatagctggtggacacagggggacagtggacaaggcactcccgtggcaccagtccacgcactggctcaggcttacttcacttgaacatggctgaggatcctgcaaacaacccctgatatgtgcatgtcccagcagactgcgctggcactcagaggcccagcggggccacgtccgcctcccgttacgggcaggcccccatgctgctttgcttgatggagagagatgccctgtccacgcctgtgggtccctctacccacggcccacccacagatgtggatgacccaaagcagatgtctggatgccagtggagaggggaccagggtgtcctgcagacatgcttgagctgcagggggtctgagtcaagccctcctggcagccacaggagccctctctgtctttcagagtcaccactcccacataaagacacattctctgtctctgggtagactccagagggatgcagtcacaagtttgggcaggtaacaagggggacccttggtcttcagcaccagcaagcagaaacagagaggtcacgtcacgctgatgcttaagatggggcactggctctgggggtgtcggctcctctccctctggacgtagggctgatggcagagaaaggctctggcctcccagcgtggctcagctcggctccctcaactctgctcctcagaagtgatggccggccttcactgcctcgatgtctgagatcagcgtccttgccaggaagatgccaaatatctgcaacagcgagatggcgatgaagacgccagccacaatgtaaatgttccgcgggagccagctttccagcgcctggatgcagcctttcgtgaagatggactcatcccacttgctcttcagctgaatcctgacatcatatccacactgtgtgttcacaactttttgcgcaggatctggcacgcagcaggagaaggggaccccgcacttctctcggctgtagctggcaccgctgcaattgaagtagacgttgaggtcccagtcttcagggccatatgcgccacagcactggttagctttctgaagggagtcgatgaggttttgcagatcgatatcgtcccggtaggacttgatgttgctctcgaagaactcccggaaccggtccctcacccagtcctggaacaggaaggccagcacggccacagccagctccaggaagaagatgagcacgatggtgccacagaaaaagttgagcaagcagatattctcccgcagagcccccacgcagccggcgaaccccagggtgaacatcaccacgcccaccatcaggaccagcaccacagggtcgattccatgcatccgggtcactttggtgaggtcggacagcacacccttttcgctccatgcccacagcccgactccaaggaagacaactccagccaaccagaagatgatgttgtagctgaaaaggaggtacttgtaccagcagctgaccttggcgttagagtatctataatagtgcatcttctgagaagcagaatcttgttaacaatgcaaactctgattcagctgatctggatggagacccctcaagattctacagcgcagcaagctcccaggtgatgctcatgctgcccatcagcaggtctgtggatggcactttgaatagtaaggatgtaacgcaactcacagggctccctgctttcgactccaccccaagtcccgcgcgcggcggcggcagcggcggcgcggcccggctcggccgaggaagttagagcaagttc

SEQ ID NO: 11067 - RNA, 5700 nt, Homo sapiens
  source 1..5700: mol_type = other RNA
ctgaatagctgggactacaggtgcacatcaccatgcccgactaatttttgtatttttagtagaaactgggtatcaccatgttgtccaggctggtctcgaactcctggcctcaagtgatctgcctgtcttagcctcccaaagttctgggattacaggcgtgagccactgcacctggccagttctagtagttattaaaccatgcattggaagaccctgctggaatataagatgcagagcacagaaagaaaactaagtgaagaaagaattgtttcggagccttgtaaggaatactcacgtcctccttctccaagctgggctccctgaagttggcaatttcatcaaaacagtatccacttaaaagtacccttaactttttcttccaaagttacacagtagccccaagttctacaatgcccacttcatgttttcctgaggcaccctggagacgccaaaagcatttgagaatgaacgggcctttttttttttttttttttcttttttgagcccaggctggagtgcagtggtgtgatctcggctcactgcaagctccgcctcctgggttcacaccattcccctgcctcagcctccggagtagctgggactacaggcacccgccaccaagcccggctaatttttttgtatttttagtagagaaggggtttcaccgtattagccaggatggtgaacatgcctttaatgcagccttgaacaggaattggccaagccttgccaacttgataaggagcaaaaaaggctctaaaggtgtatggctccccagatttctggagggcatccaaatgaatgagaacagggctgcaggtagtcacctgcagcatcctcctgggcacgatgacagagggaagtgtctctaccaagatccatcatgggggacaggttcccatagccccggacacacaacctaaaaaccgtggttctgtggaccgacacccgtaagaccctagagctggaaaggcccacctgtgaaggtcattcagcactccaccacccaccccctaccagtacagctgaaagctctggaccagcgggtgacaggctgatgcatctgacatttgggcggagaccttcccatgacagcaggatgcctcaggtgctgggaccactgctgcctccctcctttctcagcagtcgtctatgttcctctgagactgctggctgagaagccatcaggtgggttccctgatgagactgacaccctctctgctctgctgggagccttccaacactgcagccacctacagtcacatgcatgcctgccacctccccagtggcctctgcatggaatctcccagagaaattccacgttccaggaaggttgtgcatccattaattttcattgttattcatggggaaacccagtgccaggcttcttgtggaccatgcagatggtttttcagcccagcccacagccctgccctgtgggtagtgggattccccggaggctggtgaggacagctgcagcagagtcctaagcagacatatgggagaggtcagagaactggcgagcctgggcctctgaagcagagaagcagaggacattcaggaggtgcagtgtctggtgctacagaggctgaagaaggccagagttgacaattgggataagcagctttcagctacgtggggcatggtgggtggtgcaaaggaaggggtacagacagcccagataagaagctgcctgggaaagaaagggagggagccatagggcctcggcaagtttttaggatgggaaaggaaggccagcgataggaagacgggacaggaaaaataacgttgacaagatcctgagagggggtggaccagggttgaggagggggtacaggaaagaccccaaggctttaaagttagcatgtgcatggtgaggtgagaagagggtgcaaatgccacagctggcctccaaccagggaaggcggggattcaggacaggccagtgctaggtggggagtgcacaggaggcctgccctgtgcctctgtgcggacagccgatgctgggcggagactgccacgtgaccggctctcatccttgctttctttccattcctcatccaactattcagagtcacatgatatggctgagaacagccagaagggtctatagttgaaagataaacccaactctgcaaaaatcgcaccgagacttcatcctaaaccaggtctacaggaatagatgggtcaggcctgcaggagccttccaggagctctggcagggagggtctgtggccacccactcccccaggggaggctgggtcagaggcatctagtgaggtgggcactgccaccaacccccttcacagaaaggccggcacacccaggacacacagctcatgcagcagcagtgcccaggcttcaatcccatgtccccacttcgactcagtgtccccaagctcttctgcttggatcaataaatagtatcgcacaggggtggacagaaataacctaaaacaatgtttcctctagacctatggagttgaagtttctccagctctcacttatagcgggggataaaccacaagccaacttgtgcggctgtggccggcacacaagggcaactgaaagtgctgccatacagaatcttaaaaaaaaaaaaaattactcaatgaaatgtaagtcagattgtgctgatgatggactgcctttaccatccatccttctgtaaggtctacataccctatcccttggttcctctggcagccgcgtttaccactgagatgcttagcaatatctcaatagtgaccccaaacaaaaatgaccaaaacagcattaatataaagatatattccataaaagagtttggcagtcaaagagaagcatcacacttccgaaaaacacaagcattcttctcctagtctacagagaattgtgtaaaaaaaaaaaaatcatcatcaacagccaccagtatacaccacactagaatgtacactccggcaagtaaattaaggttgcagtccatccctgaacgatgagaagtggtctgagctatggcaaagtgttagaaagtagcccagctagacaaatgccccagctatccccaggggagttattcagtacttaagacttcatttccaagagcagccccagaaaagccctgacaggaagggtggaccagtgatcaccgatatcccattaggggcggtcaccagaaacaaaatgcctggagcttctgagcagctgcagcctggggttgtggctaggcacggggtgtggttgcagaagaacggctgtctccggggagaggcaaatggcaggccagccagccctgggtacatggccacaagaggagccctggccaacagtttcaggctggccatcttgggctggggctccctgggcttgcagtggggagggtcaggattcaaattctgggtgacaatttcagtagcaccaagaccagaagacagtgaggccacgctggggagtgggggagtgcttgtatgtgggatgcatggagggaggctgcagtatgtggaggagaaagagaggctgttgtgggctggttcttaagacactcaaggggactcaaagggtcggctccagccatggacactatctaaggctgctcagaggagaatgctggaggagaggaagaggaagtgaaatggtgtgagaacattcttacccctataaataaactatttacacactttaagaaaaggagagccggctctcagtgaagaaccatgcccaccgcgccaccggcgccatcagggcttaatgctatcaagaccagaggcagttccggcgccaggagaatagctggtggacacagggggacagtggacaaggcactcccgtggcaccagtccacgcactggctcaggcttacttcacttgaacatggctgaggatcctgcaaacaacccctgatatgtgcatgtcccagcagactgcgctggcactcagaggcccagcggggccacgtccgcctcccgttacgggcaggcccccatgctgctttgcttgatggagagagatgccctgtccacgcctgtgggtccctctacccacggcccacccacagatgtggatgacccaaagcagatgtctggatgccagtggagaggggaccagggtgtcctgcagacatgcttgagctgcagggggtctgagtcaagccctcctggcagccacaggagccctctctgtctttcagagtcaccactcccacataaagacacattctctgtctctgggtagactccagagggatgcagtcacaagtttgggcaggtaacaagggggacccttggtcttcagcaccagcaagcagaaacagagaggtcacgtcacgctgatgcttaagatggggcactggctctgggggtgtcggctcctctccctctggacgtagggctgatggcagagaaaggctctggcctcccagcgtggctcagctcggctccctcaactctgctcctcagaagtgatggccggccttcactgcctcgatgtctgagatcagcgtccttgccaggaagatgccaaatatctgcaacagcgagatggcgatgaagacgccagccacaatgtaaatgttccgcgggagccagctttccagcgcctggatgcagcctttcgtgaagatggactcatcccacttgctcttcagctgaatcctgacatcatatccacactgtgtgttcacaactttttgcgcaggatctggcacgcagcaggagaaggggaccccgcacttctctcggctgtagctggcaccgctgcaattgaagtagacgttgaggtcccagtcttcagggccatatgcgccacagcactggttagctttctgaagggagtcgatgaggttttgcagatcgatatcgtcccggtaggacttgatgttgctctcgaagaactcccggaaccggtccctcacccagtcctggaacaggaaggccagcacggccacagccagctccaggaagaagatgagcacgatggtgccacagaaaaagttgagcaagcagatattctcccgcagagcccccacgcagccggcgaaccccagggtgaacatcaccacgcccaccatcaggaccagcaccacagggtcgattccatgcatccgggtcactttggtgaggtcggacagcacacccttttcgctccatgcccacagcccgactccaaggaagacaactccagccaaccagaagatgatgttgtagctgaaaaggaggtacttgtaccagcagctgaccttggcgttagagtatctataatagtgcatcttctgagaagcagaatcttgttaacaatgcaaactctgattcagctgatctggatggagacccctcaagattctacagcgcagcaagctcccaggtgatgctcatgctgcccatcagcaggtctgtggatggcactttgaatagtaaggatgtaacgccatgcaggacagcccaactccagctctcccaaatgccaggaaacacaaagactctgaggcagcaccaggagctcacctcttaccagaatcccagaagccactttagagacaactgccccagctctcaggctcccagctcaggccagcacagcctaaggagggaggagccagttcctccagctatctagctgaaaggcacaggctctaggccttctccctggctgctcagttgggaggcagtacagaccgcaaggggtgaagagtttcaaccccagcctgcccaggcccacttaagctct

SEQ ID NO: 11068 - RNA, 5462 nt, Homo sapiens
  source 1..5462: mol_type = other RNA
ctgaatagctgggactacaggtgcacatcaccatgcccgactaatttttgtatttttagtagaaactgggtatcaccatgttgtccaggctggtctcgaactcctggcctcaagtgatctgcctgtcttagcctcccaaagttctgggattacaggcgtgagccactgcacctggccagttctagtagttattaaaccatgcattggaagaccctgctggaatataagatgcagagcacagaaagaaaactaagtgaagaaagaattgtttcggagccttgtaaggaatactcacgtcctccttctccaagctgggctccctgaagttggcaatttcatcaaaacagtatccacttaaaagtacccttaactttttcttccaaagttacacagtagccccaagttctacaatgcccacttcatgttttcctgaggcaccctggagacgccaaaagcatttgagaatgaacgggcctttttttttttttttttttcttttttgagcccaggctggagtgcagtggtgtgatctcggctcactgcaagctccgcctcctgggttcacaccattcccctgcctcagcctccggagtagctgggactacaggcacccgccaccaagcccggctaatttttttgtatttttagtagagaaggggtttcaccgtattagccaggatggtgaacatgcctttaatgcagccttgaacaggaattggccaagccttgccaacttgataaggagcaaaaaaggctctaaaggtgtatggctccccagatttctggagggcatccaaatgaatgagaacagggctgcaggtagtcacctgcagcatcctcctgggcacgatgacagagggaagtgtctctaccaagatccatcatgggggacaggttcccatagccccggacacacaacctaaaaaccgtggttctgtggaccgacacccgtaagaccctagagctggaaaggcccacctgtgaaggtcattcagcactccaccacccaccccctaccagtacagctgaaagctctggaccagcgggtgacaggctgatgcatctgacatttgggcggagaccttcccatgacagcaggatgcctcaggtgctgggaccactgctgcctccctcctttctcagcagtcgtctatgttcctctgagactgctggctgagaagccatcaggtgggttccctgatgagactgacaccctctctgctctgctgggagccttccaacactgcagccacctacagtcacatgcatgcctgccacctccccagtggcctctgcatggaatctcccagagaaattccacgttccaggaaggttgtgcatccattaattttcattgttattcatggggaaacccagtgccaggcttcttgtggaccatgcagatggtttttcagcccagcccacagccctgccctgtgggtagtgggattccccggaggctggtgaggacagctgcagcagagtcctaagcagacatatgggagaggtcagagaactggcgagcctgggcctctgaagcagagaagcagaggacattcaggaggtgcagtgtctggtgctacagaggctgaagaaggccagagttgacaattgggataagcagctttcagctacgtggggcatggtgggtggtgcaaaggaaggggtacagacagcccagataagaagctgcctgggaaagaaagggagggagccatagggcctcggcaagtttttaggatgggaaaggaaggccagcgataggaagacgggacaggaaaaataacgttgacaagatcctgagagggggtggaccagggttgaggagggggtacaggaaagaccccaaggctttaaagttagcatgtgcatggtgaggtgagaagagggtgcaaatgccacagctggcctccaaccagggaaggcggggattcaggacaggccagtgctaggtggggagtgcacaggaggcctgccctgtgcctctgtgcggacagccgatgctgggcggagactgccacgtgaccggctctcatccttgctttctttccattcctcatccaactattcagagtcacatgatatggctgagaacagccagaagggtctatagttgaaagataaacccaactctgcaaaaatcgcaccgagacttcatcctaaaccaggtctacaggaatagatgggtcaggcctgcaggagccttccaggagctctggcagggagggtctgtggccacccactcccccaggggaggctgggtcagaggcatctagtgaggtgggcactgccaccaacccccttcacagaaaggccggcacacccaggacacacagctcatgcagcagcagtgcccaggcttcaatcccatgtccccacttcgactcagtgtccccaagctcttctgcttggatcaataaatagtatcgcacaggggtggacagaaataacctaaaacaatgtttcctctagacctatggagttgaagtttctccagctctcacttatagcgggggataaaccacaagccaacttgtgcggctgtggccggcacacaagggcaactgaaagtgctgccatacagaatcttaaaaaaaaaaaaaattactcaatgaaatgtaagtcagattgtgctgatgatggactgcctttaccatccatccttctgtaaggtctacataccctatcccttggttcctctggcagccgcgtttaccactgagatgcttagcaatatctcaatagtgaccccaaacaaaaatgaccaaaacagcattaatataaagatatattccataaaagagtttggcagtcaaagagaagcatcacacttccgaaaaacacaagcattcttctcctagtctacagagaattgtgtaaaaaaaaaaaaatcatcatcaacagccaccagtatacaccacactagaatgtacactccggcaagtaaattaaggttgcagtccatccctgaacgatgagaagtggtctgagctatggcaaagtgttagaaagtagcccagctagacaaatgccccagctatccccaggggagttattcagtacttaagacttcatttccaagagcagccccagaaaagccctgacaggaagggtggaccagtgatcaccgatatcccattaggggcggtcaccagaaacaaaatgcctggagcttctgagcagctgcagcctggggttgtggctaggcacggggtgtggttgcagaagaacggctgtctccggggagaggcaaatggcaggccagccagccctgggtacatggccacaagaggagccctggccaacagtttcaggctggccatcttgggctggggctccctgggcttgcagtggggagggtcaggattcaaattctgggtgacaatttcagtagcaccaagaccagaagacagtgaggccacgctggggagtgggggagtgcttgtatgtgggatgcatggagggaggctgcagtatgtggaggagaaagagaggctgttgtgggctggttcttaagacactcaaggggactcaaagggtcggctccagccatggacactatctaaggctgctcagaggagaatgctggaggagaggaagaggaagtgaaatggtgtgagaacattcttacccctataaataaactatttacacactttaagaaaaggagagccggctctcagtgaagaaccatgcccaccgcgccaccggcgccatcagggcttaatgctatcaagaccagaggcagttccggcgccaggagaatagctggtggacacagggggacagtggacaaggcactcccgtggcaccagtccacgcactggctcaggcttacttcacttgaacatggctgaggatcctgcaaacaacccctgatatgtgcatgtcccagcagactgcgctggcactcagaggcccagcggggccacgtccgcctcccgttacgggcaggcccccatgctgctttgcttgatggagagagatgccctgtccacgcctgtgggtccctctacccacggcccacccacagatgtggatgacccaaagcagatgtctggatgccagtggagaggggaccagggtgtcctgcagacatgcttgagctgcagggggtctgagtcaagccctcctggcagccacaggagccctctctgtctttcagagtcaccactcccacataaagacacattctctgtctctgggtagactccagagggatgcagtcacaagtttgggcaggtaacaagggggacccttggtcttcagcaccagcaagcagaaacagagaggtcacgtcacgctgatgcttaagatggggcactggctctgggggtgtcggctcctctccctctggacgtagggctgatggcagagaaaggctctggcctcccagcgtggctcagctcggctccctcaactctgctcctcagaagtgatggccggccttcactgcctcgatgtctgagatcagcgtccttgccaggaagatgccaaatatctgcaacagcgagatggcgatgaagacgccagccacaatgtaaatgttccgcgggagccagctttccagcgcctggatgcagcctttcgtgaagatggactcatcccacttgctcttcagctgaatcctgacatcatatccacactgtgtgttcacaactttttgcgcaggatctggcacgcagcaggagaaggggaccccgcacttctctcggctgtagctggcaccgctgcaattgaagtagacgttgaggtcccagtcttcagggccatatgcgccacagcactggttagctttctgaagggagtcgatgaggttttgcagatcgatatcgtcccggtaggacttgatgttgctctcgaagaactcccggaaccggtccctcacccagtcctggaacaggaaggccagcacggccacagccagctccaggaagaagatgagcacgatggtgccacagaaaaagttgagcaagcagatattctcccgcagagcccccacgcagccggcgaaccccagggtgaacatcaccacgcccaccatcaggaccagcaccacagggtcgattccatgcatccgggtcactttggtgaggtcggacagcacacccttttcgctccatgcccacagcccgactccaaggaagacaactccagccaaccagaagatgatgttgtagctgaaaaggaggtacttgtaccagcagctgaccttggcgttagagtatctataatagtgcatcttctgagaagcagaatcttgttaacaatgcaaactctgattcagctgatctggatggagacccctcaagattctacagcgcagcaagctcccaggtgatgctcatgctgcccatcagcaggtctgtggatggcactttgaatagtaaggatgtaacgccgcgcgcggcggcggcagcggcggcgcggcccggctcggccgaggaagttagagcaagttc

SEQ ID NO: 11069 - RNA, 5484 nt, Homo sapiens
  source 1..5484: mol_type = other RNA
ctgaatagctgggactacaggtgcacatcaccatgcccgactaatttttgtatttttagtagaaactgggtatcaccatgttgtccaggctggtctcgaactcctggcctcaagtgatctgcctgtcttagcctcccaaagttctgggattacaggcgtgagccactgcacctggccagttctagtagttattaaaccatgcattggaagaccctgctggaatataagatgcagagcacagaaagaaaactaagtgaagaaagaattgtttcggagccttgtaaggaatactcacgtcctccttctccaagctgggctccctgaagttggcaatttcatcaaaacagtatccacttaaaagtacccttaactttttcttccaaagttacacagtagccccaagttctacaatgcccacttcatgttttcctgaggcaccctggagacgccaaaagcatttgagaatgaacgggcctttttttttttttttttttcttttttgagcccaggctggagtgcagtggtgtgatctcggctcactgcaagctccgcctcctgggttcacaccattcccctgcctcagcctccggagtagctgggactacaggcacccgccaccaagcccggctaatttttttgtatttttagtagagaaggggtttcaccgtattagccaggatggtgaacatgcctttaatgcagccttgaacaggaattggccaagccttgccaacttgataaggagcaaaaaaggctctaaaggtgtatggctccccagatttctggagggcatccaaatgaatgagaacagggctgcaggtagtcacctgcagcatcctcctgggcacgatgacagagggaagtgtctctaccaagatccatcatgggggacaggttcccatagccccggacacacaacctaaaaaccgtggttctgtggaccgacacccgtaagaccctagagctggaaaggcccacctgtgaaggtcattcagcactccaccacccaccccctaccagtacagctgaaagctctggaccagcgggtgacaggctgatgcatctgacatttgggcggagaccttcccatgacagcaggatgcctcaggtgctgggaccactgctgcctccctcctttctcagcagtcgtctatgttcctctgagactgctggctgagaagccatcaggtgggttccctgatgagactgacaccctctctgctctgctgggagccttccaacactgcagccacctacagtcacatgcatgcctgccacctccccagtggcctctgcatggaatctcccagagaaattccacgttccaggaaggttgtgcatccattaattttcattgttattcatggggaaacccagtgccaggcttcttgtggaccatgcagatggtttttcagcccagcccacagccctgccctgtgggtagtgggattccccggaggctggtgaggacagctgcagcagagtcctaagcagacatatgggagaggtcagagaactggcgagcctgggcctctgaagcagagaagcagaggacattcaggaggtgcagtgtctggtgctacagaggctgaagaaggccagagttgacaattgggataagcagctttcagctacgtggggcatggtgggtggtgcaaaggaaggggtacagacagcccagataagaagctgcctgggaaagaaagggagggagccatagggcctcggcaagtttttaggatgggaaaggaaggccagcgataggaagacgggacaggaaaaataacgttgacaagatcctgagagggggtggaccagggttgaggagggggtacaggaaagaccccaaggctttaaagttagcatgtgcatggtgaggtgagaagagggtgcaaatgccacagctggcctccaaccagggaaggcggggattcaggacaggccagtgctaggtggggagtgcacaggaggcctgccctgtgcctctgtgcggacagccgatgctgggcggagactgccacgtgaccggctctcatccttgctttctttccattcctcatccaactattcagagtcacatgatatggctgagaacagccagaagggtctatagttgaaagataaacccaactctgcaaaaatcgcaccgagacttcatcctaaaccaggtctacaggaatagatgggtcaggcctgcaggagccttccaggagctctggcagggagggtctgtggccacccactcccccaggggaggctgggtcagaggcatctagtgaggtgggcactgccaccaacccccttcacagaaaggccggcacacccaggacacacagctcatgcagcagcagtgcccaggcttcaatcccatgtccccacttcgactcagtgtccccaagctcttctgcttggatcaataaatagtatcgcacaggggtggacagaaataacctaaaacaatgtttcctctagacctatggagttgaagtttctccagctctcacttatagcgggggataaaccacaagccaacttgtgcggctgtggccggcacacaagggcaactgaaagtgctgccatacagaatcttaaaaaaaaaaaaaattactcaatgaaatgtaagtcagattgtgctgatgatggactgcctttaccatccatccttctgtaaggtctacataccctatcccttggttcctctggcagccgcgtttaccactgagatgcttagcaatatctcaatagtgaccccaaacaaaaatgaccaaaacagcattaatataaagatatattccataaaagagtttggcagtcaaagagaagcatcacacttccgaaaaacacaagcattcttctcctagtctacagagaattgtgtaaaaaaaaaaaaatcatcatcaacagccaccagtatacaccacactagaatgtacactccggcaagtaaattaaggttgcagtccatccctgaacgatgagaagtggtctgagctatggcaaagtgttagaaagtagcccagctagacaaatgccccagctatccccaggggagttattcagtacttaagacttcatttccaagagcagccccagaaaagccctgacaggaagggtggaccagtgatcaccgatatcccattaggggcggtcaccagaaacaaaatgcctggagcttctgagcagctgcagcctggggttgtggctaggcacggggtgtggttgcagaagaacggctgtctccggggagaggcaaatggcaggccagccagccctgggtacatggccacaagaggagccctggccaacagtttcaggctggccatcttgggctggggctccctgggcttgcagtggggagggtcaggattcaaattctgggtgacaatttcagtagcaccaagaccagaagacagtgaggccacgctggggagtgggggagtgcttgtatgtgggatgcatggagggaggctgcagtatgtggaggagaaagagaggctgttgtgggctggttcttaagacactcaaggggactcaaagggtcggctccagccatggacactatctaaggctgctcagaggagaatgctggaggagaggaagaggaagtgaaatggtgtgagaacattcttacccctataaataaactatttacacactttaagaaaaggagagccggctctcagtgaagaaccatgcccaccgcgccaccggcgccatcagggcttaatgctatcaagaccagaggcagttccggcgccaggagaatagctggtggacacagggggacagtggacaaggcactcccgtggcaccagtccacgcactggctcaggcttacttcacttgaacatggctgaggatcctgcaaacaacccctgatatgtgcatgtcccagcagactgcgctggcactcagaggcccagcggggccacgtccgcctcccgttacgggcaggcccccatgctgctttgcttgatggagagagatgccctgtccacgcctgtgggtccctctacccacggcccacccacagatgtggatgacccaaagcagatgtctggatgccagtggagaggggaccagggtgtcctgcagacatgcttgagctgcagggggtctgagtcaagccctcctggcagccacaggagccctctctgtctttcagagtcaccactcccacataaagacacattctctgtctctgggtagactccagagggatgcagtcacaagtttgggcaggtaacaagggggacccttggtcttcagcaccagcaagcagaaacagagaggtcacgtcacgctgatgcttaagatggggcactggctctgggggtgtcggctcctctccctctggacgtagggctgatggcagagaaaggctctggcctcccagcgtggctcagctcggctccctcaactctgctcctcagaagtgatggccggccttcactgcctcgatgtctgagatcagcgtccttgccaggaagatgccaaatatctgcaacagcgagatggcgatgaagacgccagccacaatgtaaatgttccgcgggagccagctttccagcgcctggatgcagcctttcgtgaagatggactcatcccacttgctcttcagctgaatcctgacatcatatccacactgtgtgttcacaactttttgcgcaggatctggcacgcagcaggagaaggggaccccgcacttctctcggctgtagctggcaccgctgcaattgaagtagacgttgaggtcccagtcttcagggccatatgcgccacagcactggttagctttctgaagggagtcgatgaggttttgcagatcgatatcgtcccggtaggacttgatgttgctctcgaagaactcccggaaccggtccctcacccagtcctggaacaggaaggccagcacggccacagccagctccaggaagaagatgagcacgatggtgccacagaaaaagttgagcaagcagatattctcccgcagagcccccacgcagccggcgaaccccagggtgaacatcaccacgcccaccatcaggaccagcaccacagggtcgattccatgcatccgggtcactttggtgaggtcggacagcacacccttttcgctccatgcccacagcccgactccaaggaagacaactccagccaaccagaagatgatgttgtagctgaaaaggaggtacttgtaccagcagctgaccttggcgttagagtatctataatagtgcatcttctgagaagcagaatcttgttaacaatgcaaactctgattcagctgatctggatggagacccctcaagattctacagcgcagcaagctcccaggtgatgctcatgctgcccatcagcaggtctgtggatggcactttgaatagtaaggatgtaacgctcttccaagaccaccgccctcctgtgttcgtgccggcagaaacacagcctagagcagtgacacaggctggccccgaagacaat

SEQ ID NO: 11070 - RNA, 5488 nt, Homo sapiens
  source 1..5488: mol_type = other RNA
ctgaatagctgggactacaggtgcacatcaccatgcccgactaatttttgtatttttagtagaaactgggtatcaccatgttgtccaggctggtctcgaactcctggcctcaagtgatctgcctgtcttagcctcccaaagttctgggattacaggcgtgagccactgcacctggccagttctagtagttattaaaccatgcattggaagaccctgctggaatataagatgcagagcacagaaagaaaactaagtgaagaaagaattgtttcggagccttgtaaggaatactcacgtcctccttctccaagctgggctccctgaagttggcaatttcatcaaaacagtatccacttaaaagtacccttaactttttcttccaaagttacacagtagccccaagttctacaatgcccacttcatgttttcctgaggcaccctggagacgccaaaagcatttgagaatgaacgggcctttttttttttttttttttcttttttgagcccaggctggagtgcagtggtgtgatctcggctcactgcaagctccgcctcctgggttcacaccattcccctgcctcagcctccggagtagctgggactacaggcacccgccaccaagcccggctaatttttttgtatttttagtagagaaggggtttcaccgtattagccaggatggtgaacatgcctttaatgcagccttgaacaggaattggccaagccttgccaacttgataaggagcaaaaaaggctctaaaggtgtatggctccccagatttctggagggcatccaaatgaatgagaacagggctgcaggtagtcacctgcagcatcctcctgggcacgatgacagagggaagtgtctctaccaagatccatcatgggggacaggttcccatagccccggacacacaacctaaaaaccgtggttctgtggaccgacacccgtaagaccctagagctggaaaggcccacctgtgaaggtcattcagcactccaccacccaccccctaccagtacagctgaaagctctggaccagcgggtgacaggctgatgcatctgacatttgggcggagaccttcccatgacagcaggatgcctcaggtgctgggaccactgctgcctccctcctttctcagcagtcgtctatgttcctctgagactgctggctgagaagccatcaggtgggttccctgatgagactgacaccctctctgctctgctgggagccttccaacactgcagccacctacagtcacatgcatgcctgccacctccccagtggcctctgcatggaatctcccagagaaattccacgttccaggaaggttgtgcatccattaattttcattgttattcatggggaaacccagtgccaggcttcttgtggaccatgcagatggtttttcagcccagcccacagccctgccctgtgggtagtgggattccccggaggctggtgaggacagctgcagcagagtcctaagcagacatatgggagaggtcagagaactggcgagcctgggcctctgaagcagagaagcagaggacattcaggaggtgcagtgtctggtgctacagaggctgaagaaggccagagttgacaattgggataagcagctttcagctacgtggggcatggtgggtggtgcaaaggaaggggtacagacagcccagataagaagctgcctgggaaagaaagggagggagccatagggcctcggcaagtttttaggatgggaaaggaaggccagcgataggaagacgggacaggaaaaataacgttgacaagatcctgagagggggtggaccagggttgaggagggggtacaggaaagaccccaaggctttaaagttagcatgtgcatggtgaggtgagaagagggtgcaaatgccacagctggcctccaaccagggaaggcggggattcaggacaggccagtgctaggtggggagtgcacaggaggcctgccctgtgcctctgtgcggacagccgatgctgggcggagactgccacgtgaccggctctcatccttgctttctttccattcctcatccaactattcagagtcacatgatatggctgagaacagccagaagggtctatagttgaaagataaacccaactctgcaaaaatcgcaccgagacttcatcctaaaccaggtctacaggaatagatgggtcaggcctgcaggagccttccaggagctctggcagggagggtctgtggccacccactcccccaggggaggctgggtcagaggcatctagtgaggtgggcactgccaccaacccccttcacagaaaggccggcacacccaggacacacagctcatgcagcagcagtgcccaggcttcaatcccatgtccccacttcgactcagtgtccccaagctcttctgcttggatcaataaatagtatcgcacaggggtggacagaaataacctaaaacaatgtttcctctagacctatggagttgaagtttctccagctctcacttatagcgggggataaaccacaagccaacttgtgcggctgtggccggcacacaagggcaactgaaagtgctgccatacagaatcttaaaaaaaaaaaaaattactcaatgaaatgtaagtcagattgtgctgatgatggactgcctttaccatccatccttctgtaaggtctacataccctatcccttggttcctctggcagccgcgtttaccactgagatgcttagcaatatctcaatagtgaccccaaacaaaaatgaccaaaacagcattaatataaagatatattccataaaagagtttggcagtcaaagagaagcatcacacttccgaaaaacacaagcattcttctcctagtctacagagaattgtgtaaaaaaaaaaaaatcatcatcaacagccaccagtatacaccacactagaatgtacactccggcaagtaaattaaggttgcagtccatccctgaacgatgagaagtggtctgagctatggcaaagtgttagaaagtagcccagctagacaaatgccccagctatccccaggggagttattcagtacttaagacttcatttccaagagcagccccagaaaagccctgacaggaagggtggaccagtgatcaccgatatcccattaggggcggtcaccagaaacaaaatgcctggagcttctgagcagctgcagcctggggttgtggctaggcacggggtgtggttgcagaagaacggctgtctccggggagaggcaaatggcaggccagccagccctgggtacatggccacaagaggagccctggccaacagtttcaggctggccatcttgggctggggctccctgggcttgcagtggggagggtcaggattcaaattctgggtgacaatttcagtagcaccaagaccagaagacagtgaggccacgctggggagtgggggagtgcttgtatgtgggatgcatggagggaggctgcagtatgtggaggagaaagagaggctgttgtgggctggttcttaagacactcaaggggactcaaagggtcggctccagccatggacactatctaaggctgctcagaggagaatgctggaggagaggaagaggaagtgaaatggtgtgagaacattcttacccctataaataaactatttacacactttaagaaaaggagagccggctctcagtgaagaaccatgcccaccgcgccaccggcgccatcagggcttaatgctatcaagaccagaggcagttccggcgccaggagaatagctggtggacacagggggacagtggacaaggcactcccgtggcaccagtccacgcactggctcaggcttacttcacttgaacatggctgaggatcctgcaaacaacccctgatatgtgcatgtcccagcagactgcgctggcactcagaggcccagcggggccacgtccgcctcccgttacgggcaggcccccatgctgctttgcttgatggagagagatgccctgtccacgcctgtgggtccctctacccacggcccacccacagatgtggatgacccaaagcagatgtctggatgccagtggagaggggaccagggtgtcctgcagacatgcttgagctgcagggggtctgagtcaagccctcctggcagccacaggagccctctctgtctttcagagtcaccactcccacataaagacacattctctgtctctgggtagactccagagggatgcagtcacaagtttgggcaggtaacaagggggacccttggtcttcagcaccagcaagcagaaacagagaggtcacgtcacgctgatgcttaagatggggcactggctctgggggtgtcggctcctctccctctggacgtagggctgatggcagagaaaggctctggcctcccagcgtggctcagctcggctccctcaactctgctcctcagaagtgatggccggccttcactgcctcgatgtctgagatcagcgtccttgccaggaagatgccaaatatctgcaacagcgagatggcgatgaagacgccagccacaatgtaaatgttccgcgggagccagctttccagcgcctggatgcagcctttcgtgaagatggactcatcccacttgctcttcagctgaatcctgacatcatatccacactgtgtgttcacaactttttgcgcaggatctggcacgcagcaggagaaggggaccccgcacttctctcggctgtagctggcaccgctgcaattgaagtagacgttgaggtcccagtcttcagggccatatgcgccacagcactggttagctttctgaagggagtcgatgaggttttgcagatcgatatcgtcccggtaggacttgatgttgctctcgaagaactcccggaaccggtccctcacccagtcctggaacaggaaggccagcacggccacagccagctccaggaagaagatgagcacgatggtgccacagaaaaagttgagcaagcagatattctcccgcagagcccccacgcagccggcgaaccccagggtgaacatcaccacgcccaccatcaggaccagcaccacagggtcgattccatgcatccgggtcactttggtgaggtcggacagcacacccttttcgctccatgcccacagcccgactccaaggaagacaactccagccaaccagaagatgatgttgtagctgaaaaggaggtacttgtaccagcagctgaccttggcgttagagtatctataatagtgcatcttctgagaagcagaatcttgttaacaatgcaaactctgattcagctgatctggatggagacccctcaagattctacagcgcagcaagctcccaggtgatgctcatgctgcccatcagcaggtctgtggatggcactttgaatagtaaggatgtaacgctgcctcttccaagaccaccgccctcctgtgttcgtgccggcagaaacacagcctagagcagtgacacaggctggccccgaagacaat

SEQ ID NO: 11071 - RNA, 4952 nt, Homo sapiens
  source 1..4952: mol_type = other RNA
ctgaatagctgggactacaggtgcacatcaccatgcccgactaatttttgtatttttagtagaaactgggtatcaccatgttgtccaggctggtctcgaactcctggcctcaagtgatctgcctgtcttagcctcccaaagttctgggattacaggcgtgagccactgcacctggccagttctagtagttattaaaccatgcattggaagaccctgctggaatataagatgcagagcacagaaagaaaactaagtgaagaaagaattgtttcggagccttgtaaggaatactcacgtcctccttctccaagctgggctccctgaagttggcaatttcatcaaaacagtatccacttaaaagtacccttaactttttcttccaaagttacacagtagccccaagttctacaatgcccacttcatgttttcctgaggcaccctggagacgccaaaagcatttgagaatgaacgggcctttttttttttttttttttcttttttgagcccaggctggagtgcagtggtgtgatctcggctcactgcaagctccgcctcctgggttcacaccattcccctgcctcagcctccggagtagctgggactacaggcacccgccaccaagcccggctaatttttttgtatttttagtagagaaggggtttcaccgtattagccaggatggtgaacatgcctttaatgcagccttgaacaggaattggccaagccttgccaacttgataaggagcaaaaaaggctctaaaggtgtatggctccccagatttctggagggcatccaaatgaatgagaacagggctgcaggtagtcacctgcagcatcctcctgggcacgatgacagagggaagtgtctctaccaagatccatcatgggggacaggttcccatagccccggacacacaacctaaaaaccgtggttctgtggaccgacacccgtaagaccctagagctggaaaggcccacctgtgaaggtcattcagcactccaccacccaccccctaccagtacagctgaaagctctggaccagcgggtgacaggctgatgcatctgacatttgggcggagaccttcccatgacagcaggatgcctcaggtgctgggaccactgctgcctccctcctttctcagcagtcgtctatgttcctctgagactgctggctgagaagccatcaggtgggttccctgatgagactgacaccctctctgctctgctgggagccttccaacactgcagccacctacagtcacatgcatgcctgccacctccccagtggcctctgcatggaatctcccagagaaattccacgttccaggaaggttgtgcatccattaattttcattgttattcatggggaaacccagtgccaggcttcttgtggaccatgcagatggtttttcagcccagcccacagccctgccctgtgggtagtgggattccccggaggctggtgaggacagctgcagcagagtcctaagcagacatatgggagaggtcagagaactggcgagcctgggcctctgaagcagagaagcagaggacattcaggaggtgcagtgtctggtgctacagaggctgaagaaggccagagttgacaattgggataagcagctttcagctacgtggggcatggtgggtggtgcaaaggaaggggtacagacagcccagataagaagctgcctgggaaagaaagggagggagccatagggcctcggcaagtttttaggatgggaaaggaaggccagcgataggaagacgggacaggaaaaataacgttgacaagatcctgagagggggtggaccagggttgaggagggggtacaggaaagaccccaaggctttaaagttagcatgtgcatggtgaggtgagaagagggtgcaaatgccacagctggcctccaaccagggaaggcggggattcaggacaggccagtgctaggtggggagtgcacaggaggcctgccctgtgcctctgtgcggacagccgatgctgggcggagactgccacgtgaccggctctcatccttgctttctttccattcctcatccaactattcagagtcacatgatatggctgagaacagccagaagggtctatagttgaaagataaacccaactctgcaaaaatcgcaccgagacttcatcctaaaccaggtctacaggaatagatgggtcaggcctgcaggagccttccaggagctctggcagggagggtctgtggccacccactcccccaggggaggctgggtcagaggcatctagtgaggtgggcactgccaccaacccccttcacagaaaggccggcacacccaggacacacagctcatgcagcagcagtgcccaggcttcaatcccatgtccccacttcgactcagtgtccccaagctcttctgcttggatcaataaatagtatcgcacaggggtggacagaaataacctaaaacaatgtttcctctagacctatggagttgaagtttctccagctctcacttatagcgggggataaaccacaagccaacttgtgcggctgtggccggcacacaagggcaactgaaagtgctgccatacagaatcttaaaaaaaaaaaaaattactcaatgaaatgtaagtcagattgtgctgatgatggactgcctttaccatccatccttctgtaaggtctacataccctatcccttggttcctctggcagccgcgtttaccactgagatgcttagcaatatctcaatagtgaccccaaacaaaaatgaccaaaacagcattaatataaagatatattccataaaagagtttggcagtcaaagagaagcatcacacttccgaaaaacacaagcattcttctcctagtctacagagaattgtgtaaaaaaaaaaaaatcatcatcaacagccaccagtatacaccacactagaatgtacactccggcaagtaaattaaggttgcagtccatccctgaacgatgagaagtggtctgagctatggcaaagtgttagaaagtagcccagctagacaaatgccccagctatccccaggggagttattcagtacttaagacttcatttccaagagcagccccagaaaagccctgacaggaagggtggaccagtgatcaccgatatcccattaggggcggtcaccagaaacaaaatgcctggagcttctgagcagctgcagcctggggttgtggctaggcacggggtgtggttgcagaagaacggctgtctccggggagaggcaaatggcaggccagccagccctgggtacatggccacaagaggagccctggccaacagtttcaggctggccatcttgggctggggctccctgggcttgcagtggggagggtcaggattcaaattctgggtgacaatttcagtagcaccaagaccagaagacagtgaggccacgctggggagtgggggagtgcttgtatgtgggatgcatggagggaggctgcagtatgtggaggagaaagagaggctgttgtgggctggttcttaagacactcaaggggactcaaagggtcggctccagccatggacactatctaaggctgctcagaggagaatgctggaggagaggaagaggaagtgaaatggtgtgagaacattcttacccctataaataaactatttacacactttaagaaaaggagagccggctctcagtgaagaaccatgcccaccgcgccaccggcgccatcagggcttaatgctatcaagaccagaggcagttccggcgccaggagaatagctggtggacacagggggacagtggacaaggcactcccgtggcaccagtccacgcactggctcaggcttacttcacttgaacatggctgaggatcctgcaaacaacccctgatatgtgcatgtcccagcagactgcgctggcactcagaggcccagcggggccacgtccgcctcccgttacgggcaggcccccatgctgctttgcttgatggagagagatgccctgtccacgcctgtgggtccctctacccacggcccacccacagatgtggatgacccaaagcagatgtctggatgccagtggagaggggaccagggtgtcctgcagacatgcttgagctgcagggggtctgagtcaagccctcctggcagccacaggagccctctctgtctttcagagtcaccactcccacataaagacacattctctgtctctgggtagactccagagggatgcagtcacaagtttgggcaggtaacaagggggacccttggtcttcagcaccagcaagcagaaacagagaggtcacgtcacgctgatgcttaagatggggcactggctctgggggtgtcggctcctctccctctggacgtagggctgatggcagagaaaggctctggcctcccagcgtggctcagctcggctccctcaactctgctcctcagaagtgatggccggccttcactgcctcgatgtctgagatcagcgtccttgccaggaagatgccaaatatctgcaacagcgagatggcgatgaagacgccagccacaatgtaaatgttccgcgggagccagctttccagcgcctggatgcagcctttcgtgaagatggactcatcccacttgctcttcagctgaatcctgacatcatatccacactgtgtgttcacaactttttgcgcaggatctggcacgcagcaggagaaggggaccccgcacttctctcggctgtagctggcaccgctgcaattgaagtagacgttgaggtcccagtcttcagggccatatgcgccacagcactggttccagaagatgatgttgtagctgaaaaggaggtacttgtaccagcagctgaccttggcgttagagtatctataatagtgcatcttctgagaagcagaatccgcgcgcggcggcggcagcggcggcgcggcccggctcggccgaggaagttagagcaagttc

SEQ ID NO: 11072 - RNA, 1728 nt, Homo sapiens
  source 1..1728: mol_type = other RNA
ctgaatagctgggactacaggtgcacatcaccatgcccggctaatttttttgtgtattttgtacaggcaggatctcatcatgttgcccaagctggcctcaaactcctgggctcaagcaaaccacccaccttggcttcccatagtgctgggattacaggcatgagccaccatacctggccaacatatcatacttttaaagtacttttaaatatagtacatttcccttgtaattcctttatataataagtccacctatgtgcattagtaagcttctttacaactcacctccaaatttaaagaattaattcatgcattggcttacagcaaaagaacttttgttttgattcatgtgtttaaaagaagaaatcaattaaagttcaattttaatatccaaagatgtaaggtggcaaatgttaccttctcaaggaagttttttctaccttcaagttcacagaaaatcataaaatgaaaacaatcactaggcataaatcagttataaagctacctttctaacacaatgcagctcactacatactccacaaaggtgaagtaaataacatcaaactcaaattttatcttgataactacacagtaatttttgctaattatatagcttaatttccaaatcttttcacatcattttaaaatatattctacatttctgagttttgatttgacaaaatggtaatcatttaaaatgaccctacttaaaaaaaaaattacaatttacaatttacaatcacttaaacaccaggatctaagttaaaacattagcaggcttcttgctctactttttacatttttatactaaacatatcccttaagtaaggatctacatttccatgttgtaataaaacattcagttacttaaattaagcagtgggggcatttatctgcaataagaagttacacaattacagtgctcatgtgcataaagtgatgatgctttcccaagcagctcatagacagaaacacagaaacactttttaaacatatttgttgatgaccctaaagacacacacttctaagtgtttgctttggaataaatgaacagccagcattttacttatcaagaaaccccaaggctttattagtattagaaatcagtaaagaaatccaaaactaaagaaaaacaaaaacgcctttttaaaaatacaacttcccttgttaagtgtattaatgcagtttttgtgtacctttgaaaattcttcaggttcctttatatctaatgaccttgttgcaaattctaatagttcttcagagttctccagggcattattacattgactaatctgactctgtaactcttgggatttacgagcttgttcctgcttgatacagttaatcatactttcttttacttcatccagtatagagtataaactatcaaattcttcatctaactctgagagtatgttggacgaattttcctgaactccttttagtgtatgatgtagtgtatcaataaagttctgaatttcatcatttttatttgccagagttgaaatgatcctctgtagagcttctttctgggagtccatggcgagtggctaagcccactgggctcgaacccgagacgacgaaccgtgtgaggaggctcagcgagatcgcacaccccaagaccgctactcactgcactgccccagcccgcaccggcaccgcccggccccacccgtccgcgcccagaccgcgcgcgccgtagtcacgccgcggttgccagggtgaaag

SEQ ID NO: 11073 - RNA, 1088 nt, Homo sapiens
  source 1..1088: mol_type = other RNA
ctgaatagctgggactacaggtgcacatcgccacgcctaacttttttatttttagtacagatgggagcctcactatattgcccagactgccttggcctcccaaagtactgggattacaagcgtgagccaccatccccagccaagcacttctttaggaaagattattgctttgggcaagctgaaggttgggtccgggagcgtggtcactgcctgaggccactcagcgaccagatgccggatttgaaccgctgtgattctaacagcggagcctgcacatgcgcactctaggggcctgggctctttgctcaccaacagccgggatcaagttgaaggtcttaagcctagaggtggcctccacgatgctctgtggcatctcctcgtgtgttaagtccacgaggagtacggagtccccccagcggcggtagtgcgccagctctgtcaggtactgtgggtctccggtgggcagctctagggagtccatgatgtgcaggtcgtcctgggccagcttgacggtcagtgccactttgagacccagcgcccgcaccttcatgggcagcatgtagtagtaacttgtggggccccgggggccatgggcaacacctcctcctcgccagagcggagagcggatgctgccatgccgggcccgcccagtgcctttctgcggccaaggcttccggccaccgccccgcacctcggctctcgtcttggtcttggcatagctaattctcttgaagttcttctgccacatagcaacctggtgcagtatgtccagcctgggcgcggtggcgaaaacatcggggtgcaggtcggccaggcccacgcgctcctgctcgaagccccgcaaggactcgacccaggcctgcactgggcgtcgatgagtgggtaccgggagctcgactttgcgcagcacgggctccgggagaccctcgctcgccacctgctccgggttctcggtcgcacgcgctgcctcttccgccagggaactcaggccctggctgccggtaggccgaagccaggcccgcgccccggcccggacgaactgcagcatcgccgcgcagcctcccacgccgcgggaggtcaaggccact

SEQ ID NO: 11074 - RNA, 3343 nt, Homo sapiens
  source 1..3343: mol_type = other RNA
ctgaatagctgggactacaggtgcaccaccatgcccagctaaatttttgtatttttagtagagatggggtttcaccatgctggccaggctggtcttgaactcctgatctcatgatctgcctgccttggcctcccaaagtgctgggattataggtgtgagccaccgcacccagccatctgatggtttttttaaattgagaaataaaatgaataaccataatgaatactaagatgacaattttttgaggggggatactagaaaagtttcaagaacatacaaggaactcacatacccctttacacagaaggatcaattgtttgtattttgcctcatttacttgatgagttattctcatctttctctctctggatctgtctgacatatatacatcactatttcttttccttgaatcatttgagaataagttataaccatgcccctttattcctaaatactcctgtgttaattcctaagaacaggggtccccagattgtgcgctccttatgagaatctaatgcctgatgatctgaggtggaacagtttcatcctgaaaccatccccccaacccaggtctgcggaaaaattttcttccaggaaactggtccctggtgccaaaaaggttgggaactgctgcctaagaacaaggccattctcttacatgatcacaagccaattatcaacttcaggaaatgttaatgttaatacaataccttcatctcatttactatccacatccaatgttgccatttggcccgatgatgtcttttatagcctgacccactatgttttcatggctgaatgcatattaagaattaatataagtaattaagaattaataatgagtagagtgctttggcatttagaaagcccttttgctacattaactcatttgcttctcactttgcctctctgaggtcaggcagcagctctatccttggtttacccaagatagaaatgaggttgaggggacatcaaatccaaagcagtgctcagacctcattcttccctcacaccactggttggtgttcattttaaagactttatttgtcttagtgccaaccagcagactgactactaacccagatattttattttgtgagacagggtctcttgctctgacttccaggctggagtgcagtggcatgatcttggctcactgtagcctcagcctcctgggctcacgtgatcctcctgcctcagcctcctgcggaattgggaccgcaggtgtgcaccaccacacctggctaatttcttgattttctgaagagatgaggtctcactatgttgcccaggctggtctcaaactcctgggctcaagcaaccctccagtctcccaaagtgctgggactacaggcagagccacctcacctagccccctcaaatattttaaattccaaaaataaacgaatatagttcaagtgcttgtctctctaaccaaaaacaaatgaatatcgtttgggtgctgttgcttcatgttagcaacacagattctaattatcacctgcggctacacatgcaggaagagtcctgaactccccagggtctgagagcttggtatcagctgggaggcccctgatgggcaagtaggggggcctggcttccttggtgcccacccagcctgttttgtggagcccaccccaccatgcatgccgaacttgaacccacaactggcaaaaaatccccaatcccaggcttgacttgaacatagaaagccgagacacactggggatctcttccagggcacagtgaaacgttggtttgggggcagagaggcagtttctcaatcctcagtagtagccttttccaaggcctctctgtcaagcagttcttgcacagctagaagcttgatgctgttttccaggagtgtcatgcacaccacctctcgcaccccggggttgttggccttctccacggaacagccctgcaagttccaggtggccagcctcagcacaggcctcccatcccttgtgcctccaaaggcctccacggacggccgagtggagataatctgggtgggcccccctggcggcaggtccaggtcctcactctgcaggctcagggaagtggggctcgggtgaggcttggcggtgaaggtcagtcccccgttcgtgtgggtggatgggggcctggacctctcagcaaacacctggtgccggatcctgtccaggaaggcggcattgataccatccatcctcactaggtcctcaacgctgcgaaagggcccatgctcacggcggaagtccacgatgctgagggccattttctccgagaggcctcgcacgctcatgagctgggccggggtggctgtgttgatgttaacacgtggggtgaggggcacagctgtggccaggtggtgaggctgctgctccgctagcaggtcccgccgcagggaactgggagagtgctgcgctgagctgcccttgctgctcacacagatctcaaacttgacctgctccagcttggtggcgcctacaccactgaccaatgccaggtcctccaccttcttgaagccaccgatatactctcggtactccacgatgctgcgtgccacggcacgcgtcaccccaggcagggtcatcagctcctcctccgtggcagtgttgatgttgagccgctcctgattcactagaatgttgctgaagttacaggctgcgctgaacttgcggctatgggacaggtccgaggggtccctggggatggagcggtggcagcccagggtgctccccatggtccgccaggatcaggctcccgggaaggccgcaccactgcagaagagctctctggctagggaggaagcccagtaggccgtacaagcacagaaaaacggaaggtgcaggattcagggactgaagaggttactatagacaaacaccgaatcttccatgcctggcgtgtccaaaattacctttcacttggccgcctctcggccgctctgcggggcgccggttcctcttccacctgcggctcggaagcctgagcccagcccgggacagcacgggccccctgcctccagcctaggcgtccgcgcgggtgtgggtcactggtcaggccctggaagccgactacgccgcttcggtctgcgtgtcccggctctttctatgggagaaacttagcatcgctctcccagagtgaatagaagccgcagggctgctcggaggcggcggcagcggcggcgaaacccgccgccgaggctgcaccggggcttgcggcggcgccgccgcagttgcgtttaccccggcaaaaagtcctgcgcccaactcgggcggggatccgccagagccagtccagacccagcaccagccgcacggctcccgctcgcagtcggtgtcaaagccaaagtccc

SEQ ID NO: 11075 - RNA, 4018 nt, Homo sapiens
  source 1..4018: mol_type = other RNA
ctgaatagctgggactacaggtgcaccccaccacacctggcatttttgttgttgttgcccaagctggtctcaaacccctgggctcaagcaaccctcccacctcagcctcccaaagtgctgggagtacaggcacgagccatcaggcttggccaaataagcgtttattggacagatccagttctccaaagtttagagcaggttaacttggtagctatggagtatgaccagatggagacatgggtcttgtggccggccctgcgactggctgacagtccagcaaggcaaggaggtaggtacttcacacactgtgcacacccatctcaggcagccgtagacccctacgcctccccaccccacaggcacatgcaggctccagggaaagcaagtagttggcaggtgcctctccaacctggtgtctttgggcatccttgccctgggcgacacagtgagaccctgtctcaaaaaaagtccctcccatgccagctgcctgtgtcccaaccactcaggtgctttgcctctcaacagaatccacctgcagttccctgctaggtatgtctcaaggagccctctagccacccgacttgtctttaatgcctataaaatccagttcagaggaggaaaaatatttatcaggcaagtcctgcctttggaggtatgtacaggcactgacatcagaacagggcagtgagtaaacccggcaccgaacaggccatcagaatagggagccccacatggtaaatgtggctgcgcatagcaagctcacccagggaaggctgggctgcaggttggggtaaagcccttgatgcaggctgtaacatgttttgatgcagaagttattggttctgagtagaaagggcaaggtaagagagcaaagcctaaaaatgcagtttcccccttgagttcttttctctcctcttatttgacttccctcccatgataacatgccccaagggctgagagccactatactgtgtttaacagatggagagaataccttctttaggctttcagagctacagaagctggggctaaaatgccaactctatagccatgaggatctgctttctttttttttttttgagacggagtctcgctctgtcacccaggctggagtgcagtggcactatctgagctcactgcaacctctgcctcccaggttcaagtgattctcgtgtctcagcttcctgagtagctgggatacaggcaagcgtcaccacacccagctaattttttgtatttttagtagagacattttaattatgttggccaggctggtctcaaacttctgacttcaggtgatccgcctgcctcagcctcccaaagtgctgggattacaggcgtgagccactgcacctggccaaggaccagcttgtgagtctagggaacctggaatgcagcagccccaatcttgactttagttaacctgtgtcatatgcaggggctttaaaggtggccaggagcagggcatctggctatctggctatctccaggtagtgggtcggggaggctctgagactgctacagagcagaccattgacagcctgtaactgagtccaaattcattctgcttgctgcgtcatagccaatacgttgagagacaaggagttggagcaaggaaagggactttatttcggagagccagcaaaccaagaagatggtggactaatgtcctaaagaaccgtcttaaaattatgcgggctttgccttgtcttttatgtttaggtcgggggaaaggaaggggctgacaaccgcagacatctggacaccagcaagggtccaggggaggtttgcagaacttctttgtccttggctaacagtctgtcatgtgacaatagccaaacctcctcattcctataaatctttaacaaaaacagttagctgtttacatgcttcccctttaatcccagagttagttttgcaaacggcatgattcctgtttttgcgttttatgtcagtgctctaaagttatcctagcctaggtgcaggaataggtaaaggccccttaaacaaaaatggagttagttatgttagttcttctgctgtttcatggttacaagacacagaagagaacccttgcatcaaaacaggatgagattaggttgttgttcctataaaaaatccatgtggttgttttttggccccctcttcaatattcggggtgtgctgacgaagcgagcagcagctctggagccataaaccaccatctcatctcagcccagggcatgctgggagaggccaggaaaagtcacttctcttctttgctttaactgtcttttctgtggcctcaaagtcttcaaaggggagacttggtgttctcagcactgctcagcctccatgaagccctccttctcatggcccgagggctccacctccgcataggtggaatggtcagggtggctgcgaaacttcatggctggccagtggtgaggtctacgctcgatgaagaagagcgcagcattggatgtggggtggccattgatgtaaattccagccaggatgatggccgccacgaggaggactgccagcacgatgcccacgatggtgcccaggtgcacaggagtgccctttgtcttgggggacaggttgttctgaaggccgtctcctcctgcatagggattcaacttggtgtcatcttctgtggtgaggctgtcgatgaagagggaggaggaggtagtggtgaggtctccatcataggggctgaaggaagtgtcaggggaggctgagtcgtggtcctcatcctggaagtcctcgcacatcctgccctctgcctcctgtgcacagccatagtccatccactcctggcgatagcggtcaaagccactggagcatctctggaggacatggcaccagctgcagttgaaggtcaggtctgaggacatgcaggcgtcacagctcctatgctgcaggcaggtcggcaatggggtgaactccacggccgacatgctggtgaccttgctggggtccagctctatgcggtgatattcaaagatgctccttcgccgagattctggcacatccggggatggattgagaatcatgaaggcatccgataggccggttttgacaggatgctgggaggagctgatttccgggacagacatagggatctctttataggcaaagacaatgcggccgtcatggtgcagagctgcctggaaggtgaaactgcccttgtcttcccagccttggagataaacgtggtcccactgaaccacaaagactgtcccattgtcaaagtaaacaactgtggagttgtcggagtagccagggttgaagttggccatcaggggcgccacatactgagtagctgtgagcatccgatggatcacgtcccccatgaagatgaagcctccagttgctatggtgatctgccgcagaggatgcccgtagaaagggaaatcaaaggacaagaccactctcgaagcctgccggtgggtgttggagagtattgtgtggatcttcacttggctccggttggcctcggccacatctacccacagttcccggctgtggggctcgctggggccatagagacgggacacataatagctgtggttgtcctccaccaccctggtcctgttatctggcagcgtgtccatggccagggtgcccccacccaggtcctggctcagctgggtcctgtccggctctgacacatgcccagggctctctcgggctctccggttccagccccgcacggtccctttggcagcccatccagagcctgggccctcatcgtgacctgctccgggctgggggctcagcgcccgggcagcctccctgagcaccagcaccaggagccagagctcgcctcgcatggtgggtgcccggacctgcccccggcctgcttgctgccccggtcctgacgagggagggggccctggctcaggctgcggccgcgcggtccccggggctggcggaggggcgggcggcgaggagacggcggagcgcggggccgggcgagccggcaggagcggcgagagcgcgagcggagctggaggctgcggcctccgggagc

SEQ ID NO: 11076 - RNA, 27 nt, Homo sapiens
  source 1..27: mol_type = other RNA
ctgaatagctgggactacaggtgcacg

SEQ ID NO: 11077 - RNA, 6725 nt, Homo sapiens
  source 1..6725: mol_type = other RNA
ctgaatagctgggactacaggtgcacgccaccaaacctggctatttttttttttttgtagagatggggggggggtctcaccatgttgcccaggctggtcttgaactcctggcctcagctgattctcctgcctcagcctccctaagtgctgggattacaggcaggagccaccatgcccagccagtttatggtaatttgctgcaaccacaggcaattaatatacactgttagcatggtccacgaggccgcacctgtgtggcccctgttaaacttctgacctcttctcatccttcaccacctgaccatccccctcccctctgggcctttgcacctgctgttcctgcttcctgagatgtcctcctcccaggttacctgtctttcttcagccagatgtcaccttcttagcgaggcttccctagtcaccttctaaacagcagccctgccactccctacaccccttccctggcttcatctttctccatgcgtcaccccacctgccatactcctcatctgtctgtttccttctaccagaaggtaggtcctaagtggatgcagcatctgtgtcacacattgctgtgccctcagtgcctggaataagcatctggcatgttgtgagcattccatagatatttgttggatgaatgaatgagtgaatgaatgaatgaaatttcacagatggggagactaagaccagggaacaggaacgccttgcctaagttagggtcagcactagtcctggaatcaaacgcggcatctcctgcatctcactgtccaaaaaatgcctccactgggcagacctgggcacttttgaaatgtttatccctcaggcctgtctcaatcttagttctgccaggtaattccacaatgaccccaggcaggtgtcctgccgtcttagtgtctagcgtctgcgtcctcatctattaatggatggacggatggatggatggatggatggatggatggatggatggatggacggacggacggacgggtggacggatgaatggatggatggatggatggacggatggatgaatgtccttagttgggaaaggctcagcaggtcagaagactaggaagaaggccagagccatgagagggcttggggaaggagaggcagccaggcacacagggggctgggacacagagtctggttccaggcaagggcttgagaagccatcaggggtttatagagagaaccgactcaatcctcccttctaagaggactgtgcagacattggactgtgtggggctggggccaaggtactggggatgaagttgaatgggagagatttgagatgcgatttgggtagaaaagacaagatttactggaaaacagaatatgaggtgggtgagtgggattaaggtgggggactgaggagtctggaagagtgcccaaggggggagtaccaaggacggcaggactttcctgcatttcttaggtaccttttaggtagaagtgatggaaacccctgtgcttgcactaagcaagatgggaaactgtatggattcctatgatggaaaaatctcgggccgcagtgctccagcggtgacccggggcccggctctctttccacctcctcattctctttttctgtgttggcatcattctcaggcaggccaccccatataatgtcaaatggcacccacagccccccactggcatcctattaggacatcaaacccagcagaaagaggctttttttctaatgttttcataacaaaagtcccaggggtgcttctcattggccaagcatgggtcacatgcccaaacccaaaccagtcactgatactggggagctggagggctctggttgttaaggctgggcccatgtgtccatccttgagccatgtgggtggagagtgggggtggttccctgagggagatgaagacaatggagaggtgccgggcagacacacaggagccagcccccgcgccctgcagggctgatacgcacaggagtctctgaggtgagggcctggcagagaaggtctggtacagcgcctgcaccatctgccttggtggcccagcctcctcccttcctggtcctgatccagtgggccttgccccacgctcccgcatgggatggcagagcccagccctgtgcctccaatcagggcaagctgccaccacactgagtacctgccccaggtcctacattgcaaattccatgacttatgaccactcaaagccacaagtgctgcctggcagggtcagtgctgaggctggggctcctacctactgtctctccctccttggctgccccctagcccgcctgcctcagtgagccagagaggtcgtgcccagtttgaatgcagtcctctaggcttcagggcacctaagttcagagctcagccctccatatttccctgtgtcctggaaaggtggggccaccctacagctgtccctgagagactgcagatacctgctcagtttctctctggttccggatcttgctgtctactctgtgggattcggactttggctcaaacacctctacaccttcttctcatggtggcaagagggctgctgcagttccagcctcacttctcagcttgaaaggcagcaggaaagagcgacagccttctctgtggctcccgctctgactggaccgctttaggtcacatgctcactcctgaccctctgtggcccatgagtgcaggaggctgcttgggcaggactgaattgcatgctccaattccaaagccccatcgggggagagctaaggcgaattcccaaaccaaaaccagggctgttgctgcaaaaaggaggcctgggtgctgaggacgcaggaaacacgtccctacctagggatcatcttcaaattataagtgaggagatggccgggcatggtggctcacaccagcactttcggaggctgaggcgggagggctgcttgagtccaggagttcaggaccagcctgggtaacacagtgagatcccgtctctacaaaaacaaacaaacaaaattagccgggcatgctagtgtgcgcctgtgatcccagctactcaggaggctgaggtgggaggatcacctgaacctgggaagtcgaggctgcagtgatctgtgatcgcaccactgaactccagcctgggaaacagagtgagaccctgtctccaaaaaataaaaataaaataagtggggaaagagaggctgggctttctagtgtcaagggctgacatgtccagagtgggcccccaggtacagacagctccccaccccaggaactaagcctttctcaggtctttgagcttttacgaatgacacaggctatgagtccatttaaaaatcattttattattaacatcatcttcccatgtagccaagtgtctgtcatgtataaggaatgtcggtaaatattccatttgaagcttctttgtacatatttccctcgataaataaactctgaattcacataaaaaagttaaacttaaataactcatatttccttctcttgtaacaggcatatattggtaaaatataaatattctcggactcaggctttgttctaagtgaggacagtaattgatcacatggtacaattattgacagtaaaaccaagaaattgtcagctggtgtcctggcatggactagtgctgaggtgggagacaggaagttcacatttggtttctgggccaaagtggggcaggaggggtggtggggagaaaaggacagttgttttctttacagctctgataaaaataatctgtgctgccactgaattttaactttgaatatattcttctacatttgctgattaattccataatcattttactgaaaactcagatgtcaactaacaaaatatggcacatgatccattttgaacaatgtcaataggttcagaaactaccattgggctggcaaaaaaaacaagagaaacgcacatggcgagagcgatgattcggggttggtttggttggttcactgtggcccactgaacactcgtccctggcctcagtgtggcagattcatccccttggggcgatggcacaagccctggtgcccggcagggcctctgaggcctgagcggcaggtgaggctggcaggcgcctgctcagagcacgcgggggatgatggtgaagggcacggcggggctgctggcctccagctccaaggctgtcaggaagcactccgtagccgccgcatcgttgccctgagcttggaggacctcgcccagcccgttccagacctcgtgggctgtcgagttcacctgcaccgcgtcccggaggatcttctccgccagactgtagcggcctagctggtgaaggatcagggccagtcgctgcatgctcttcacgtgggtggggctgatggctaaggcctcttcataccaccgccgcgcctcgtccatgcttccccggagctcagcaatctggccgcgcatgtagaggacattgtgggacattgggaagaggttggcagcttcttgggtacaggctgtggcttctgcaggcttcccgatgccgatatagacttcagctgcatggagccagatctgtgccagcgtcatccaggggtgcagcgggccctgcttaggggcactgctctgcagagacgaagccacttccgacagtgcctgctccactcttgaggctgctaccgatgtggcatggacggagcctgtctcgggatcgctgaagtctggcaaagtaattgtattaagctgtcgtctgtcagcaatggttctatctaagaggctgctcccacgtccagaatcactggggttggtgaggttgtagcaggatttccatatctgcagcatgtgcttacaagtcagcagtgcctcgtccgggcctcggcagagtgactgcaacttcactttggaaaacagtagtatgaaattttctgggtattcactcagggccatgtcgatgatgttcagagcgtcatggtaatgcttctgtgctgacagcaggagggcaaggaggtgcagggagttggcatcgtcaccttgaagctgaagagcttggcggacataccccagagcctctgggatctgtctggagatggcaagctgcagagccaggtagaaagctgcttggtgatctgtgggtgacaggctgtgggccctctgaaatgcaagaagcgcctttctctgtaggacctcctgcatccctcgcaaagaagcgtcagtggcctgcagactgtacgtgagccccagagctaagtagcctttggccttgaactctgacgttttctctcccacatcaacgacagttttggcaaacttttcagcctcttccaaccagtgcagggagcccatgcagagcttggcagcgaggagagggatggtggcatcgtctggcttcaggcggatacactctttcagcaccttcacggcacgggcagattttccagcagccatcagggacagagcaaactggtaccacaggtggaattcctcaaaggcaaacttcatggctctttctaggcactctgacagcatctcatactggcctcttcttccaagagcaatggtgagtaagtcatagaccacagatgcactctgcagactgatgaggcggtcactcttgtgttcaggtatcctgctcagcacagcgtcccggttggccattgattcactaatcagcaataacaacagggcttcttccgtattttcttgaggacaaaaaatgttctctcctgagtagacacgggctctccgagtgagagtgtaggtttttgtgtttgctcctttgcggagaggatcgtccagaggtgactggcacggtggatcctccagagggttccagtagctctgctcacacataccccgcaacaagatctctgccagctgcctggctattgtcattcgcaggttttgagtcgttcttgtttcaactgctctgagaagctctctaaatcttccgactcctcttgtcaagttcccatttttgaaatagaggacatgggctctctgaagtcctgtttctaggaaaaaacctagttcttgatcgtggggagcagggccaggcttagggcttctgttttgaatattagaaagtattaccctttctatctcttggagatacaggagtgcgatgtcccctgctttctcataacaggtgatgacatcctgttcccggtccacatggagattactggtagaagaagaaataggcagcttctccaaacaaagtcctttggtagcgtaggcttctgcgatcacccgcagcctgtagggcgggacagctgtcagtggcagatcgtccaggcccacccgggcgtaaatgttcagagcttctttataatcaccttccacataattcaacttggccatgatcagattggattcttgtaggaattctgacttaaggttccctcggtccagggcggcggtcagatgcttgcggacctcagtcagctggggcttggggcctcggggactggccccctgcctcagggggtgttccttcaggtactgctccagcttcgactccccgaggagaagctctgccatgtcatcgttggcgatgagcttggccgacagctgcttgacgagctcagggatccgctcccactggcactcggagcggcagcgctcgatctccgtctccagccgcgagcctgccttcttggtcgccatcgcggcctggccgggcccggccgcccgccccgcaggccccaccgccgccgccgcggcgccccctcgccgcctcccgccgccgccgcgggctcgggctccggctcccggctccgcggcgtaacgggagcgccggct

SEQ ID NO: 11078 - RNA, 6772 nt, Homo sapiens
  source 1..6772: mol_type = other RNA
ctgaatagctgggactacaggtgcacgccaccaaacctggctatttttttttttttgtagagatggggggggggtctcaccatgttgcccaggctggtcttgaactcctggcctcagctgattctcctgcctcagcctccctaagtgctgggattacaggcaggagccaccatgcccagccagtttatggtaatttgctgcaaccacaggcaattaatatacactgttagcatggtccacgaggccgcacctgtgtggcccctgttaaacttctgacctcttctcatccttcaccacctgaccatccccctcccctctgggcctttgcacctgctgttcctgcttcctgagatgtcctcctcccaggttacctgtctttcttcagccagatgtcaccttcttagcgaggcttccctagtcaccttctaaacagcagccctgccactccctacaccccttccctggcttcatctttctccatgcgtcaccccacctgccatactcctcatctgtctgtttccttctaccagaaggtaggtcctaagtggatgcagcatctgtgtcacacattgctgtgccctcagtgcctggaataagcatctggcatgttgtgagcattccatagatatttgttggatgaatgaatgagtgaatgaatgaatgaaatttcacagatggggagactaagaccagggaacaggaacgccttgcctaagttagggtcagcactagtcctggaatcaaacgcggcatctcctgcatctcactgtccaaaaaatgcctccactgggcagacctgggcacttttgaaatgtttatccctcaggcctgtctcaatcttagttctgccaggtaattccacaatgaccccaggcaggtgtcctgccgtcttagtgtctagcgtctgcgtcctcatctattaatggatggacggatggatggatggatggatggatggatggatggatggatggacggacggacggacgggtggacggatgaatggatggatggatggatggacggatggatgaatgtccttagttgggaaaggctcagcaggtcagaagactaggaagaaggccagagccatgagagggcttggggaaggagaggcagccaggcacacagggggctgggacacagagtctggttccaggcaagggcttgagaagccatcaggggtttatagagagaaccgactcaatcctcccttctaagaggactgtgcagacattggactgtgtggggctggggccaaggtactggggatgaagttgaatgggagagatttgagatgcgatttgggtagaaaagacaagatttactggaaaacagaatatgaggtgggtgagtgggattaaggtgggggactgaggagtctggaagagtgcccaaggggggagtaccaaggacggcaggactttcctgcatttcttaggtaccttttaggtagaagtgatggaaacccctgtgcttgcactaagcaagatgggaaactgtatggattcctatgatggaaaaatctcgggccgcagtgctccagcggtgacccggggcccggctctctttccacctcctcattctctttttctgtgttggcatcattctcaggcaggccaccccatataatgtcaaatggcacccacagccccccactggcatcctattaggacatcaaacccagcagaaagaggctttttttctaatgttttcataacaaaagtcccaggggtgcttctcattggccaagcatgggtcacatgcccaaacccaaaccagtcactgatactggggagctggagggctctggttgttaaggctgggcccatgtgtccatccttgagccatgtgggtggagagtgggggtggttccctgagggagatgaagacaatggagaggtgccgggcagacacacaggagccagcccccgcgccctgcagggctgatacgcacaggagtctctgaggtgagggcctggcagagaaggtctggtacagcgcctgcaccatctgccttggtggcccagcctcctcccttcctggtcctgatccagtgggccttgccccacgctcccgcatgggatggcagagcccagccctgtgcctccaatcagggcaagctgccaccacactgagtacctgccccaggtcctacattgcaaattccatgacttatgaccactcaaagccacaagtgctgcctggcagggtcagtgctgaggctggggctcctacctactgtctctccctccttggctgccccctagcccgcctgcctcagtgagccagagaggtcgtgcccagtttgaatgcagtcctctaggcttcagggcacctaagttcagagctcagccctccatatttccctgtgtcctggaaaggtggggccaccctacagctgtccctgagagactgcagatacctgctcagtttctctctggttccggatcttgctgtctactctgtgggattcggactttggctcaaacacctctacaccttcttctcatggtggcaagagggctgctgcagttccagcctcacttctcagcttgaaaggcagcaggaaagagcgacagccttctctgtggctcccgctctgactggaccgctttaggtcacatgctcactcctgaccctctgtggcccatgagtgcaggaggctgcttgggcaggactgaattgcatgctccaattccaaagccccatcgggggagagctaaggcgaattcccaaaccaaaaccagggctgttgctgcaaaaaggaggcctgggtgctgaggacgcaggaaacacgtccctacctagggatcatcttcaaattataagtgaggagatggccgggcatggtggctcacaccagcactttcggaggctgaggcgggagggctgcttgagtccaggagttcaggaccagcctgggtaacacagtgagatcccgtctctacaaaaacaaacaaacaaaattagccgggcatgctagtgtgcgcctgtgatcccagctactcaggaggctgaggtgggaggatcacctgaacctgggaagtcgaggctgcagtgatctgtgatcgcaccactgaactccagcctgggaaacagagtgagaccctgtctccaaaaaataaaaataaaataagtggggaaagagaggctgggctttctagtgtcaagggctgacatgtccagagtgggcccccaggtacagacagctccccaccccaggaactaagcctttctcaggtctttgagcttttacgaatgacacaggctatgagtccatttaaaaatcattttattattaacatcatcttcccatgtagccaagtgtctgtcatgtataaggaatgtcggtaaatattccatttgaagcttctttgtacatatttccctcgataaataaactctgaattcacataaaaaagttaaacttaaataactcatatttccttctcttgtaacaggcatatattggtaaaatataaatattctcggactcaggctttgttctaagtgaggacagtaattgatcacatggtacaattattgacagtaaaaccaagaaattgtcagctggtgtcctggcatggactagtgctgaggtgggagacaggaagttcacatttggtttctgggccaaagtggggcaggaggggtggtggggagaaaaggacagttgttttctttacagctctgataaaaataatctgtgctgccactgaattttaactttgaatatattcttctacatttgctgattaattccataatcattttactgaaaactcagatgtcaactaacaaaatatggcacatgatccattttgaacaatgtcaataggttcagaaactaccattgggctggcaaaaaaaacaagagaaacgcacatggcgagagcgatgattcggggttggtttggttggttcactgtggcccactgaacactcgtccctggcctcagtgtggcagattcatccccttggggcgatggcacaagccctggtgcccggcagggcctctgaggcctgagcggcaggtgaggctggcaggcgcctgctcagagcacgcgggggatgatggtgaagggcacggcggggctgctggcctccagctccaaggctgtcaggaagcactccgtagccgccgcatcgttgccctgagcttggaggacctcgcccagcccgttccagacctcgtgggctgtcgagttcacctgcaccgcgtcccggaggatcttctccgccagactgtagcggcctagctggtgaaggatcagggccagtcgctgcatgctcttcacgtgggtggggctgatggctaaggcctcttcataccaccgccgcgcctcgtccatgcttccccggagctcagcaatctggccgcgcatgtagaggacattgtgggacattgggaagaggttggcagcttcttgggtacaggctgtggcttctgcaggcttcccgatgccgatatagacttcagctgcatggagccagatctgtgccagcgtcatccaggggtgcagcgggccctgcttaggggcactgctctgcagagacgaagccacttccgacagtgcctgctccactcttgaggctgctaccgatgtggcatggacggagctaactgaaaaaagggaaggaaaaccatgaaagtatgcttctggagagttgcctgtctcgggatcgctgaagtctggcaaagtaattgtattaagctgtcgtctgtcagcaatggttctatctaagaggctgctcccacgtccagaatcactggggttggtgaggttgtagcaggatttccatatctgcagcatgtgcttacaagtcagcagtgcctcgtccgggcctcggcagagtgactgcaacttcactttggaaaacagtagtatgaaattttctgggtattcactcagggccatgtcgatgatgttcagagcgtcatggtaatgcttctgtgctgacagcaggagggcaaggaggtgcagggagttggcatcgtcaccttgaagctgaagagcttggcggacataccccagagcctctgggatctgtctggagatggcaagctgcagagccaggtagaaagctgcttggtgatctgtgggtgacaggctgtgggccctctgaaatgcaagaagcgcctttctctgtaggacctcctgcatccctcgcaaagaagcgtcagtggcctgcagactgtacgtgagccccagagctaagtagcctttggccttgaactctgacgttttctctcccacatcaacgacagttttggcaaacttttcagcctcttccaaccagtgcagggagcccatgcagagcttggcagcgaggagagggatggtggcatcgtctggcttcaggcggatacactctttcagcaccttcacggcacgggcagattttccagcagccatcagggacagagcaaactggtaccacaggtggaattcctcaaaggcaaacttcatggctctttctaggcactctgacagcatctcatactggcctcttcttccaagagcaatggtgagtaagtcatagaccacagatgcactctgcagactgatgaggcggtcactcttgtgttcaggtatcctgctcagcacagcgtcccggttggccattgattcactaatcagcaataacaacagggcttcttccgtattttcttgaggacaaaaaatgttctctcctgagtagacacgggctctccgagtgagagtgtaggtttttgtgtttgctcctttgcggagaggatcgtccagaggtgactggcacggtggatcctccagagggttccagtagctctgctcacacataccccgcaacaagatctctgccagctgcctggctattgtcattcgcaggttttgagtcgttcttgtttcaactgctctgagaagctctctaaatcttccgactcctcttgtcaagttcccatttttgaaatagaggacatgggctctctgaagtcctgtttctaggaaaaaacctagttcttgatcgtggggagcagggccaggcttagggcttctgttttgaatattagaaagtattaccctttctatctcttggagatacaggagtgcgatgtcccctgctttctcataacaggtgatgacatcctgttcccggtccacatggagattactggtagaagaagaaataggcagcttctccaaacaaagtcctttggtagcgtaggcttctgcgatcacccgcagcctgtagggcgggacagctgtcagtggcagatcgtccaggcccacccgggcgtaaatgttcagagcttctttataatcaccttccacataattcaacttggccatgatcagattggattcttgtaggaattcttaaggttccctcggtccagggcggcggtcagatgcttgcggacctcagtcagctggggcttggggcctcggggactggccccctgcctcagggggtgttccttcaggtactgctccagcttcgactccccgaggagaagctctgccatgtcatcgttggcgatgagcttggccgacagctgcttgacgagctcagggatccgctcccactggcactcggagcggcagcgctcgatctccgtctccagccgcgagcctgccttcttggtcgccatcgcggcctggccgggcccggccgcccgccccgcaggccccaccgccgccgccgcggcgccccctcgccgcctcccgccgccgccgcgggctcgggctccggctcccggctccgcggcgtaacgggagcgccggct

SEQ ID NO: 11079 - RNA, 674 nt, Homo sapiens
  source 1..674: mol_type = other RNA
ctgaatagctgggactacaggtgcacgccaccacacccggcatgggctgatcctcatcagtgggattgggaagcaggtaaagaatacagtgccgaggagaaagggcttcctcccccacacatcagacagggcaccaatgagtggggcactcaaaaaagagagcaggccctttacaccttgaatgagaccattcatgaggaatgtgtgttgagaaaatgtttcatgtagaacagtcaacattggagttgtcaaaaggccccacgcaaagaattcaaggaagatgacaatagcagcatggtacacacttggtgggccaaagccttgtagccaggtgctccccgcggcctgcgcgcccgcgcgcttctccggcatggctcccgcctcgggctccgacgccgccttctcctccagctccggcggcggctccacgctcatgccgcggccatgcccgcgccagctcggggcgctccgggacgacggcgacgccgcggaggcggcggcggtgcccgcgccctcatgggctctgcggcccgcggcggcctgcgggtcaggcggcggcgccgagggctgaggaggcggcggaggctgaagctgcggatcaggctagcagaagaccgcagctccaggaaccgaccacttagcaaaccgcaccgaccccgactgtcgcagttacc

SEQ ID NO: 11080 - RNA, 3591 nt, Homo sapiens
  source 1..3591: mol_type = other RNA
ctgaatagctgggactacaggtgcacgccaccacacctggctaattttttgtatttttagtagagacggggtttcatcatattggtgaggctggtctcaaactcctgacctcaggtgatccacccacctcggcctcccaaagtgctaggattacaggcatgagccacagcgcctggcctgggacacacatttttggacaaaaacaatgataaattctgatgctaccaaattgccttcttatgaaaaaggaatgtggcagataagacagtagctctagaacaaaccctcatgttgacaataactgggcctagggaaaaggaggcggccccttacaactcaatccatgccttcagttgtccttatcctggttcccacacttaaccacagttgacacgggcgtgatcagacatattttgttcttgttttcaagctaagcacccttgagcccctctgaaatgtcagctgcctcaaggataagggactttactgtcaacatgatgggttgggtgagggggaaggggaacaattatccaatgtttcaacaaatctcagtagtaccccaagacatagtatttttggatagccttttaactagaacagtgagcatcaaggctagtagaatagataacaccttgatgaacacacttcctggtgatgataaaagttaggagagactctccattataaatgtgttggtgccactcagaatgaaagctattgagcagaggacttggtaccctggaacaccacacttggctctgagccataccttagccaccaaggagccttcaatcgctccctgattggaagcccaggtaatgtgttaccatgataatttcattttaactcgacattcagaagtccagcttgacttgaggatggagttttacttctatccatgagggctggctttggaatgcctcccctgtgagcacagaaggatttttaacagcatctcatgcccagcgtttttgtactttccgccatccgtgctaagtagaaggcaagttctgaatgagagtgctgacagttcctcttcctgagtgggagaaagcaccacttcagtggcagagtaggacttcccaaaatagactaagaagtagctgtaggtaaatgaattatgtgttcattcacagctttattgtttcatgccaggtccaagaatacttcaagaagtacatttttaagagttcttgagacagttgtattcaaatataaggaggcctgtgaattctctttaacaaatctacaaatatgggagagaatatgtgtgtgacatcaataaatggttaagattcctagtatagagggtgctatgtttacatttttcatctctagagttcaggtaatttttatacattaaatttggggtaagacaaaaattttgtagcctttttaatttaggggaaagtagctgttcagggtgactattatttcataaaaagtttgtgttaacctagctagtaagactctggcaggatctggcatttgctctcaggagaacaatctttgcatagcaatctcaggggtatcccagctaactgaagcctctgttaggtttggacatgcctggcataacgagatgaaaactgatcaacgtgggcatgaaatcagcgggtgtggagactgagcctttctggtgaaacagaacctgggtaccaatagcttctgtttcctacacagaaattgaatcttttggctagggtttggccaggtgccaacaaatagaaagtagaagaatgtctcaaggggaagggagatggagggggccaagaagggagataatatcgtggctgtgtttcatgggaacatagagcatttacaaagggaatgtgatttactcaaatctctatatagccccatgttcacataagcttagtgcctcatagctaactggtactcaatgagtttttgttgaatcaaactaaaccacccccattccccaaaagaaatgctacaaaagcaaacacccctgagttgtgtccagtcctattagagtcctggttaaattctattccgggggacttcgcaagtggctaaaacagcaacgatcctagaaactaagggagtcccactctttgctagctgaaacagggtctgcaatctacacgatggttttaacaccgtgttctgaaagttacagagaactcttgagtgaaggatggggcaactgccccagcagaatcataccttcttcgtgggctgctgggccttcaggacatggttgggctgattatatagggatgcttccaagacggcacctgcggctctcagccttctttaacacagccgttttgtttgggatctcttccagcccctgcccacaactactgtctggctactcacttcccaattttctagtcattggtgttcactccaggttacgagagaggagggaaggtggcaaaagagaattgctatttccaaaactttggtctgagtgggaggataaactgagtgtaaatttgtgaatttgagagaaaggcagactgcatgggttatgtaaacagcaagacaagagaagagggagacaaaaggtaagactttcttcatgtgttattcctgcaacttcctggatattaaattttggtttaatgctaaagagcaggaaccattcccaagctatgtaatcactatgaagccagatctcttttaatattatggacagtacactaatagtttccattttagaaacttcagaatgatagtgaataacattttaaaagtgtttactcttcatatccattaaaacatacacaacaatttccaactaactcttggcagctcattcaccaatagagttatctgattttttttctggcatggtatcaattctccatcaactctaacaaactgcccccaaatcacagccgtcttgtgtcaaacacctgttaatactggcaagcaccatggagtccatgtcaaagagagctaaagaagatgccaaaatatctaagctatttctacaaaaaggtggtaataattttgtatgtgaacatgttagataaaaatcactggaatcagaaacgacttcaaagcttgtatgacaatgacttgattcataggatacatacaaatgaaaccaagactgctggttagaagtgctttgatcacaatctatgtgtctctactttgcccatttcctgaacctcatcttggaagaaaaagcaggatagtaaggcatgtaaaaacacatccaacctacatttctattcttcacactgctttgtgctctctgattttaaataaaaatgcaatagctgtagggtactgggatacattaaaataattgttctgctattactcaactgagcaaaggattttaaataaggataagcataaagtatctgccaacaaccatcagtcaaggctgctaacagggcttttttcaatcttctaaagcagactaaaagttgacttgctagcaagttattaaataaaagcagagaatcctacagatagatttggaaagaccacaacaaatgcatgaggtccatgactcaacaagccctcaataaagagttaaatttaaaaaaaattgtctaaggtcttcatgacttctgtgctttacattttctcgatatttaagtg

SEQ ID NO: 11081 - RNA, 6711 nt, Homo sapiens
  source 1..6711: mol_type = other RNA
ctgaatagctgggactacaggtgcacgccaccacgaccggctaatttttgtatttttagtagagacagggtttcaccatactggtcagactggtctcgaactcctgagctcaggcaatccacccacctcggcctcccaaagtgctgggattacaggcgtaagccaccgcccctagcctaatatcaatcttcgataaagcatttgccaaattacagcaactgctctgaaagaggaattgctcttctagcattatttgaccctttttaggtatccttgaccctctttaccttaagaaatggagagttccggccgggcgcggtggctcacgcctgtaatcccagtactttgggaggctgaggtgggcagatcacgaggtcaggagatcaagaccatcctggctaagacggtgaaaccccgtctccaataaaaatacaaaaattagccaggcgtggtggcgggcgcctatagtcccagctactagggaggctgaggcaggagaatggggtgaacccgggaggcggaggttgcagtgagccgagatcgcgccactgcactccagccggggcgacagagagagactccgtctaaaaaaaaaaaaaaagaaatggagagttctactaactgtcctgtgctcccagaggggattcaatgaggatcgtaagaaggaaaacaacctgcaggggaagcagcatcttggatttcagataaagtaccaaaaaatattagctatctctttctgcagacatgcctctttctctgttaacactttcagtcattcaaaaggctattggtagaggtgcagcaaatccaagtgtagatttactgtaacagtttatttaactatgctgtattcaccaataacggcattaccaataatggcattagtgcacatcaaaagatctgaaaatgctaatgggacatttcccacaaaaggaaagaaatccaatggctcctataaagggagaatatagcaatggcaagcagaatgaaaatttctgtcaaaagaaagtacttctcaaagcaatcaggaaaaactgttcccaaattaggcctggggagccacattagccactatctcagatactgattattttgtttagccttaggggcctcaatattccccctcatctgctaaacttcaacttgtttactcacaagtctgataaattccagccaagtaaccttaacattccctatggcagtgcaaaattccagacatttgtaaacactgtaaatttcacgtttggtacatgagacagcttaccggttcatctttgattctaaaaacatagctagttcctaatctatggccatttttagcaaaggtagcatcaggatcaaaacatgcttgcacacatgcacactcatgactgggagaaccatcagaactaattgctcgttaggatatagttctgaacaatttaagcagataactgactaaatggaaaacagattcacagtatctaaagccatatatcagaaattcacataattctgaggggaaaaaactcaaatatctagttaacaattgtcttcctttcaaaagcgagtcaagaggtaacattacatagctttgtattatagatcagaagaatattcaccaatatatcaaagacttcaaaaggcagccaacattgcattgaattgacacacacaaaatgttacaaatgaccttgacccttaaaaataaattcttacaaaccaaataataccacacaatgcactacatacatctaactatacataaattataattaaaacacaactgcatatttcaaatgcttggcagtgactcaatcttacattacagaagttagtggcagtgtggaggctggcatggctcaactccaatccattgtacaagcctaggattagaaacccatactattccattggtagactggggaaatggcataccatattaaagatctggtctaagatttttataaagtttgatttaagcattaaataaaaaagcataccaattactgtgaagtacactggaaggagagtgagttaatattcagacagaagaactttttagccgtaatactgaaattcatcgttgttctaatgatttgtcatctctgctctgaacttttcgcccaagataacaatcataaatattaatttgacaactaaaacaagaaatctgatggtaatgtggtgtgatttcattattcatagtctacagcacgttgcagcagaaacaagctccaatgacacagatccttcctcacaatcaagatatcaactcgaacaaggcttacctataactaggtgaccatataatttaacatccaaatgaagaggtttgaaagtgaaaggggacatgcagaaagaaaccaggtgggatgcagaaaaatgggagcaatttggcagtctccagaaaaccagagcacatggtcccaataactacagctaaaaggtaaatgtcagtatttggaagtttccttatagcagtaaactctgaacacttcacatataaactatgccttgctttagtttagtggcagtgagtaaaaaaaatctgtaccgcagtggcaaggaaaaaagaaaatcaaaaacagaccaagaaaatagtttaagctgggcgctgtggctcatgcctgtaatctcagcactttgcgaggctgaggtgggtggatgacctgaggtcaggagttcgagaccagcctgaccaacatggtgaaaccatctctactaaaaatacaaaattagccagacatggtggtgcacacctgtaatcccagctacttgggaggctgaggcaggagaatcatttgaacccgggaggcagaggttgcagtgagccgagatcactccactgcactccagcctgggcgacaagagcaaaactccatctcaagtaaaaaaaaaaaaaaaagaaaagaaaagaaatagtttaaagtttcctacaagtaaagatgaaattcggctcaagcacatatcttaggatcgtctaagtacttagtgctaacagaagcagtgaaaaaccccggtgggcaagcaggaagagtgaagctgagcagcctaagaggattctttcatgggcaatgatgtgtcaaatttaggatcaaatacctataaacataagtaaaatgtttacttcttaagttttattaaaaattacaacttggctgggtgcggtagctcacgcctgtaatcgcaggactttgggaggccgaggtgtgtggatcatgaggtcaggagttcgagaccagcctggccaacacagtgaaacccccatctctactaaaaatacaaaaattagccaggcatggtggtatgtgcctgtagtcccagctatctgggaggctgaggcaggagaatcacctgaacccgggaggcagaggttgcggtgagcagagatcatgccattgcactccagcctgggcaacagagtgagactgtctcaaaaaaaaaaaaaaaaaccaacaacgacattatgagatttttctttttgcgattttttttttcttttttctgagacagtttcgctattgttgcccaggctggggtgcaatggcgcaatctcagctcaccgcaatctccccctctcaggttcaagcgattctcctgcctcagcctcctgagtagctgggactacaggcatgcaccaccatgcccagctaattttttgtatttttagtaaaaatggggtttctccatgtcggtcaggctggtctcaaactcccgacctaggtgatctcccaaagtgttgggattacaggcgtgagccactacgcccggtccacgattttttttttttttttttttagctcatcagctattgttagtgttagtgtattttatgtgtggtccaagacaattcttcttccattgtggaccagggaagccaaaagattggacacccctgtctagggcaaggattccaaaagtatgttctgtataaaacttgcatagagattccaggaacacttgttcaaatgcaaattcctggtccagatctcaaagatcagtctctgcacgtttggacatttttaacaagcaaccctcatgatttttatgatccttaagtttgacaattctagggccttggtcttcaaaatgacacatgcatacccttgagaacacaccaacattttcccatgggggtaaggatacatgcatagctctatggaaaccaacttaaagatgtccaatttccatatgtgttgtcctaaaatatgtgctctgatgaggcctcttcagatctaccatttctctttacctcccttttcacaacagccatactccctatcctccaaaaaaaaaaaaaaaaaaaaaaaaaaaaagaggctgcctctcaaccatccagtatatcaaggcgtattgccttggtgtaagcagctccagaggcactaaacaaaaggatcaaaaaaaatctaaatgactcctaagacgcaaagagggtagggggcagtagctcaggactgcaatcctagcactttgagaggctgaggcaggagggttgcttgaggctagaagtttgggaccagcctgggcaacatggcaaaatgctgtctgtacaaaaaatacaaaattcagctgggcatggtggtggcacgcgcctatagacccagctacttgggaggcttaggtgggaggattgcttggatctgggaggtcgaggctgcagtgaactgtgattgtgccagtgcactccagcctgggcgacagagcaagaccctgtctcaaaaaacaaaacaaaacaaaacaaaaactgatgcttctgaaggctgtgccagagaagtatgtttgtgtgtttatctgaattaaaaccaagacatgttctgacggaagttaagtctgatttggctaattaaattaagaacagactttgccagtttatatgacaggactttttctataaatttaatcagctaaatctatagtcccagggctttcataaaaatatctttgagccaagcatagtggctcaaggctgtaagcccaacactttgggaggctgaggcgggggaatcacttaaacccaggagttcgagaccagcctgggcaacataacgagacaccgtctacaaattattttaattagctgggagtgatagtgaatgcctgtgagggaagctgaggctggaggatcacttgagcccaggaggtgggccgtgtttgcaccactgcactccagcttggatgacaaagtgagaccgtctctcaaaaaaaaaaaaaaactttaaagcacatatataatatgcaatatgttggatagtatatcctttgtaagtacttaaattttaaaaatttagatttcagattaaagtcttgcaaaagggccagactaggtgcctcatgactataatcccagcaatttggaaggctgaggcgggaggattgtttgagcccaggagttcgagaccagcctgggcaacatagtgagacttcatctccacaaaaaattagccagtgtggttatgctagtctatagtctcagctactcaggaggctgaagtgggaagaccacttatgcccaggaaaccaaggctgcagtgagccatgatcataccactgcactgcacttcagcctgggagacagaacaagacagaccctgtcgccccacacctcccctatacccccggaaaaaaaaaagtgcaaaaaaaaaaaaaactagggtgagagccatgaaatagctgaaggactgtctgaagaggggcagaagggagtgttttggggtgacagaaacattctattgcttttttgggtggttactcagatttctacaactcgttagaaggaaacactttatcatgttaattatacctcaatattgtaaatgtgcatggaagaaatctcttgttttcaagagtttttcttttgggttcacctaactatgtacctgactgctgcataaagtaatccatggcacttaataatttgactaatcagattacttctgttcttcattgttagctccagtatttttcttacagctaccttggattttgatgcctaagaacattctctgacaggttggaaataaaattaaataaaggattgattttcaaataatgtggtaagtgaacggaataaatgcatttttatgttcgtactaccattatgctataaaaaccttaataaccagctgaatctctttcttgcaaatagggcatgaagccccagccttctttagtcttctggcacagtgaaaacaagtgacaagatggcccgtccttccatgaataatgttcccgtctcgtggtcttttctcacataagctacatggcttcaagagattctggcaatcctccatgttttctgtatctgttctctgttcagaaaggttatctaactgttctcccatgcttgagatggtctcttggctttcagaactgtgagccaaatccaagaattccactgagttgcagggatcaaaaagtttggagttttctttctttatatacgcatctttaggtctaacgacaggagccgaaatggttcttcgacaatcagggacatcatttccttcattttcctgattgatttgtccaggagagatcctgcaagcactgtcagatgttgaacactgagcagaggtggaaaatgatgtcattttggtagtgaagaaactgcagtctgttggtaaaacttacggcagctccatgagtcgctcccccgccgagcccgggtggggggaggggtggcagtcacagatcctagggcctcggcagcattttgaaatggcgagtaat

SEQ ID NO: 11082 - RNA, 7020 nt, Homo sapiens
  source 1..7020: mol_type = other RNA
ctgaatagctgggactacaggtgcacgccaccacgaccggctaatttttgtatttttagtagagacagggtttcaccatactggtcagactggtctcgaactcctgagctcaggcaatccacccacctcggcctcccaaagtgctgggattacaggcgtaagccaccgcccctagcctaatatcaatcttcgataaagcatttgccaaattacagcaactgctctgaaagaggaattgctcttctagcattatttgaccctttttaggtatccttgaccctctttaccttaagaaatggagagttccggccgggcgcggtggctcacgcctgtaatcccagtactttgggaggctgaggtgggcagatcacgaggtcaggagatcaagaccatcctggctaagacggtgaaaccccgtctccaataaaaatacaaaaattagccaggcgtggtggcgggcgcctatagtcccagctactagggaggctgaggcaggagaatggggtgaacccgggaggcggaggttgcagtgagccgagatcgcgccactgcactccagccggggcgacagagagagactccgtctaaaaaaaaaaaaaaagaaatggagagttctactaactgtcctgtgctcccagaggggattcaatgaggatcgtaagaaggaaaacaacctgcaggggaagcagcatcttggatttcagataaagtaccaaaaaatattagctatctctttctgcagacatgcctctttctctgttaacactttcagtcattcaaaaggctattggtagaggtgcagcaaatccaagtgtagatttactgtaacagtttatttaactatgctgtattcaccaataacggcattaccaataatggcattagtgcacatcaaaagatctgaaaatgctaatgggacatttcccacaaaaggaaagaaatccaatggctcctataaagggagaatatagcaatggcaagcagaatgaaaatttctgtcaaaagaaagtacttctcaaagcaatcaggaaaaactgttcccaaattaggcctggggagccacattagccactatctcagatactgattattttgtttagccttaggggcctcaatattccccctcatctgctaaacttcaacttgtttactcacaagtctgataaattccagccaagtaaccttaacattccctatggcagtgcaaaattccagacatttgtaaacactgtaaatttcacgtttggtacatgagacagcttaccggttcatctttgattctaaaaacatagctagttcctaatctatggccatttttagcaaaggtagcatcaggatcaaaacatgcttgcacacatgcacactcatgactgggagaaccatcagaactaattgctcgttaggatatagttctgaacaatttaagcagataactgactaaatggaaaacagattcacagtatctaaagccatatatcagaaattcacataattctgaggggaaaaaactcaaatatctagttaacaattgtcttcctttcaaaagcgagtcaagaggtaacattacatagctttgtattatagatcagaagaatattcaccaatatatcaaagacttcaaaaggcagccaacattgcattgaattgacacacacaaaatgttacaaatgaccttgacccttaaaaataaattcttacaaaccaaataataccacacaatgcactacatacatctaactatacataaattataattaaaacacaactgcatatttcaaatgcttggcagtgactcaatcttacattacagaagttagtggcagtgtggaggctggcatggctcaactccaatccattgtacaagcctaggattagaaacccatactattccattggtagactggggaaatggcataccatattaaagatctggtctaagatttttataaagtttgatttaagcattaaataaaaaagcataccaattactgtgaagtacactggaaggagagtgagttaatattcagacagaagaactttttagccgtaatactgaaattcatcgttgttctaatgatttgtcatctctgctctgaacttttcgcccaagataacaatcataaatattaatttgacaactaaaacaagaaatctgatggtaatgtggtgtgatttcattattcatagtctacagcacgttgcagcagaaacaagctccaatgacacagatccttcctcacaatcaagatatcaactcgaacaaggcttacctataactaggtgaccatataatttaacatccaaatgaagaggtttgaaagtgaaaggggacatgcagaaagaaaccaggtgggatgcagaaaaatgggagcaatttggcagtctccagaaaaccagagcacatggtcccaataactacagctaaaaggtaaatgtcagtatttggaagtttccttatagcagtaaactctgaacacttcacatataaactatgccttgctttagtttagtggcagtgagtaaaaaaaatctgtaccgcagtggcaaggaaaaaagaaaatcaaaaacagaccaagaaaatagtttaagctgggcgctgtggctcatgcctgtaatctcagcactttgcgaggctgaggtgggtggatgacctgaggtcaggagttcgagaccagcctgaccaacatggtgaaaccatctctactaaaaatacaaaattagccagacatggtggtgcacacctgtaatcccagctacttgggaggctgaggcaggagaatcatttgaacccgggaggcagaggttgcagtgagccgagatcactccactgcactccagcctgggcgacaagagcaaaactccatctcaagtaaaaaaaaaaaaaaaagaaaagaaaagaaatagtttaaagtttcctacaagtaaagatgaaattcggctcaagcacatatcttaggatcgtctaagtacttagtgctaacagaagcagtgaaaaaccccggtgggcaagcaggaagagtgaagctgagcagcctaagaggattctttcatgggcaatgatgtgtcaaatttaggatcaaatacctataaacataagtaaaatgtttacttcttaagttttattaaaaattacaacttggctgggtgcggtagctcacgcctgtaatcgcaggactttgggaggccgaggtgtgtggatcatgaggtcaggagttcgagaccagcctggccaacacagtgaaacccccatctctactaaaaatacaaaaattagccaggcatggtggtatgtgcctgtagtcccagctatctgggaggctgaggcaggagaatcacctgaacccgggaggcagaggttgcggtgagcagagatcatgccattgcactccagcctgggcaacagagtgagactgtctcaaaaaaaaaaaaaaaaaccaacaacgacattatgagatttttctttttgcgattttttttttcttttttctgagacagtttcgctattgttgcccaggctggggtgcaatggcgcaatctcagctcaccgcaatctccccctctcaggttcaagcgattctcctgcctcagcctcctgagtagctgggactacaggcatgcaccaccatgcccagctaattttttgtatttttagtaaaaatggggtttctccatgtcggtcaggctggtctcaaactcccgacctaggtgatctcccaaagtgttgggattacaggcgtgagccactacgcccggtccacgattttttttttttttttttttagctcatcagctattgttagtgttagtgtattttatgtgtggtccaagacaattcttcttccattgtggaccagggaagccaaaagattggacacccctgtctagggcaaggattccaaaagtatgttctgtataaaacttgcatagagattccaggaacacttgttcaaatgcaaattcctggtccagatctcaaagatcagtctctgcacgtttggacatttttaacaagcaaccctcatgatttttatgatccttaagtttgacaattctagggccttggtcttcaaaatgacacatgcatacccttgagaacacaccaacattttcccatgggggtaaggatacatgcatagctctatggaaaccaacttaaagatgtccaatttccatatgtgttgtcctaaaatatgtgctctgatgaggcctcttcagatctaccatttctctttacctcccttttcacaacagccatactccctatcctccaaaaaaaaaaaaaaaaaaaaaaaaaaaaagaggctgcctctcaaccatccagtatatcaaggcgtattgccttggtgtaagcagctccagaggcactaaacaaaaggatcaaaaaaaatctaaatgactcctaagacgcaaagagggtagggggcagtagctcaggactgcaatcctagcactttgagaggctgaggcaggagggttgcttgaggctagaagtttgggaccagcctgggcaacatggcaaaatgctgtctgtacaaaaaatacaaaattcagctgggcatggtggtggcacgcgcctatagacccagctacttgggaggcttaggtgggaggattgcttggatctgggaggtcgaggctgcagtgaactgtgattgtgccagtgcactccagcctgggcgacagagcaagaccctgtctcaaaaaacaaaacaaaacaaaacaaaaactgatgcttctgaaggctgtgccagagaagtatgtttgtgtgtttatctgaattaaaaccaagacatgttctgacggaagttaagtctgatttggctaattaaattaagaacagactttgccagtttatatgacaggactttttctataaatttaatcagctaaatctatagtcccagggctttcataaaaatatctttgagccaagcatagtggctcaaggctgtaagcccaacactttgggaggctgaggcgggggaatcacttaaacccaggagttcgagaccagcctgggcaacataacgagacaccgtctacaaattattttaattagctgggagtgatagtgaatgcctgtgagggaagctgaggctggaggatcacttgagcccaggaggtgggccgtgtttgcaccactgcactccagcttggatgacaaagtgagaccgtctctcaaaaaaaaaaaaaaactttaaagcacatatataatatgcaatatgttggatagtatatcctttgtaagtacttaaattttaaaaatttagatttcagattaaagtcttgcaaaagggccagactaggtgcctcatgactataatcccagcaatttggaaggctgaggcgggaggattgtttgagcccaggagttcgagaccagcctgggcaacatagtgagacttcatctccacaaaaaattagccagtgtggttatgctagtctatagtctcagctactcaggaggctgaagtgggaagaccacttatgcccaggaaaccaaggctgcagtgagccatgatcataccactgcactgcacttcagcctgggagacagaacaagacagaccctgtcgccccacacctcccctatacccccggaaaaaaaaaagtgcaaaaaaaaaaaaaactagggtgagagccatgaaatagctgaaggactgtctgaagaggggcagaagggagtgttttggggtgacagaaacattctattgcttttttgggtggttactcagatttctacaactcgttagaaggaaacactttatcatgttaattatacctcaatattgtaaatgtgcatggaagaaatctcttgttttcaagagtttttcttttgggttcacctaactatgtacctgactgctgcataaagtaatccatggcacttaataatttgactaatcagattacttctgttcttcattgttagctccagtatttttcttacagctaccttggattttgatgcctaagaacattctctgacaggttggaaataaaattaaataaaggattgattttcaaataatgtggtaagtgaacggaataaatgcatttttatgttcgtactaccattatgctataaaaaccttaataaccagctgaatctctttcttgcaaatagggcatgaagccccagccttctttagtcttctggcacagtgaaaacaagtgacaagatggcccgtccttccatgaataatgttcccgtctcgtggtcttttctcacataagctacatggcttcaagagattctggcaatcctccatgttttctgtatctgttctctgttcagaaaggttatctaactgttctcccatgcttgagatggtctcttggctttcagaactgtgagccaaatccaagaattccactgagttgcagggatcaaaaagtttggagttttctttctttatatacgcatctttaggtctaacgacaggagccgaaatggttcttcgacaatcagggacatcatttccttcattttccttttcaggtatggcagtgatatcagacgtggagagagaatgggttaactttgaacaatctgaataccaatccttcctcaaggcccaacaacgaaaacagtacctcttgcttggagagttaaatttcttgcattcagtacactgccactcatcctcagaggtaacctctacatcggtatcatcacttaaggacttagagtcctccaggtcatcattttttcccacttcaatcacctctttaacagtgaacatttcaccttgcgcacctgctgcatgcaaaatcttcaaaagcggcagttttggtcgtacctgattgatttgtccaggagagatcctgcaagcactgtcagatgttgaacactgagcagaggtggaaaatgatgtcattttggtagtgaagaaactgcagtctgttggtaaaacttacggcagctccatgagtcgctcccccgccgagcccgggtggggggaggggtggcagtcacagatcctagggcctcggcagcattttgaaatggcgagtaat

SEQ ID NO: 11083 - RNA, 7539 nt, Homo sapiens
  source 1..7539: mol_type = other RNA
ctgaatagctgggactacaggtgcacgccaccacgaccggctaatttttgtatttttagtagagacagggtttcaccatactggtcagactggtctcgaactcctgagctcaggcaatccacccacctcggcctcccaaagtgctgggattacaggcgtaagccaccgcccctagcctaatatcaatcttcgataaagcatttgccaaattacagcaactgctctgaaagaggaattgctcttctagcattatttgaccctttttaggtatccttgaccctctttaccttaagaaatggagagttccggccgggcgcggtggctcacgcctgtaatcccagtactttgggaggctgaggtgggcagatcacgaggtcaggagatcaagaccatcctggctaagacggtgaaaccccgtctccaataaaaatacaaaaattagccaggcgtggtggcgggcgcctatagtcccagctactagggaggctgaggcaggagaatggggtgaacccgggaggcggaggttgcagtgagccgagatcgcgccactgcactccagccggggcgacagagagagactccgtctaaaaaaaaaaaaaaagaaatggagagttctactaactgtcctgtgctcccagaggggattcaatgaggatcgtaagaaggaaaacaacctgcaggggaagcagcatcttggatttcagataaagtaccaaaaaatattagctatctctttctgcagacatgcctctttctctgttaacactttcagtcattcaaaaggctattggtagaggtgcagcaaatccaagtgtagatttactgtaacagtttatttaactatgctgtattcaccaataacggcattaccaataatggcattagtgcacatcaaaagatctgaaaatgctaatgggacatttcccacaaaaggaaagaaatccaatggctcctataaagggagaatatagcaatggcaagcagaatgaaaatttctgtcaaaagaaagtacttctcaaagcaatcaggaaaaactgttcccaaattaggcctggggagccacattagccactatctcagatactgattattttgtttagccttaggggcctcaatattccccctcatctgctaaacttcaacttgtttactcacaagtctgataaattccagccaagtaaccttaacattccctatggcagtgcaaaattccagacatttgtaaacactgtaaatttcacgtttggtacatgagacagcttaccggttcatctttgattctaaaaacatagctagttcctaatctatggccatttttagcaaaggtagcatcaggatcaaaacatgcttgcacacatgcacactcatgactgggagaaccatcagaactaattgctcgttaggatatagttctgaacaatttaagcagataactgactaaatggaaaacagattcacagtatctaaagccatatatcagaaattcacataattctgaggggaaaaaactcaaatatctagttaacaattgtcttcctttcaaaagcgagtcaagaggtaacattacatagctttgtattatagatcagaagaatattcaccaatatatcaaagacttcaaaaggcagccaacattgcattgaattgacacacacaaaatgttacaaatgaccttgacccttaaaaataaattcttacaaaccaaataataccacacaatgcactacatacatctaactatacataaattataattaaaacacaactgcatatttcaaatgcttggcagtgactcaatcttacattacagaagttagtggcagtgtggaggctggcatggctcaactccaatccattgtacaagcctaggattagaaacccatactattccattggtagactggggaaatggcataccatattaaagatctggtctaagatttttataaagtttgatttaagcattaaataaaaaagcataccaattactgtgaagtacactggaaggagagtgagttaatattcagacagaagaactttttagccgtaatactgaaattcatcgttgttctaatgatttgtcatctctgctctgaacttttcgcccaagataacaatcataaatattaatttgacaactaaaacaagaaatctgatggtaatgtggtgtgatttcattattcatagtctacagcacgttgcagcagaaacaagctccaatgacacagatccttcctcacaatcaagatatcaactcgaacaaggcttacctataactaggtgaccatataatttaacatccaaatgaagaggtttgaaagtgaaaggggacatgcagaaagaaaccaggtgggatgcagaaaaatgggagcaatttggcagtctccagaaaaccagagcacatggtcccaataactacagctaaaaggtaaatgtcagtatttggaagtttccttatagcagtaaactctgaacacttcacatataaactatgccttgctttagtttagtggcagtgagtaaaaaaaatctgtaccgcagtggcaaggaaaaaagaaaatcaaaaacagaccaagaaaatagtttaagctgggcgctgtggctcatgcctgtaatctcagcactttgcgaggctgaggtgggtggatgacctgaggtcaggagttcgagaccagcctgaccaacatggtgaaaccatctctactaaaaatacaaaattagccagacatggtggtgcacacctgtaatcccagctacttgggaggctgaggcaggagaatcatttgaacccgggaggcagaggttgcagtgagccgagatcactccactgcactccagcctgggcgacaagagcaaaactccatctcaagtaaaaaaaaaaaaaaaagaaaagaaaagaaatagtttaaagtttcctacaagtaaagatgaaattcggctcaagcacatatcttaggatcgtctaagtacttagtgctaacagaagcagtgaaaaaccccggtgggcaagcaggaagagtgaagctgagcagcctaagaggattctttcatgggcaatgatgtgtcaaatttaggatcaaatacctataaacataagtaaaatgtttacttcttaagttttattaaaaattacaacttggctgggtgcggtagctcacgcctgtaatcgcaggactttgggaggccgaggtgtgtggatcatgaggtcaggagttcgagaccagcctggccaacacagtgaaacccccatctctactaaaaatacaaaaattagccaggcatggtggtatgtgcctgtagtcccagctatctgggaggctgaggcaggagaatcacctgaacccgggaggcagaggttgcggtgagcagagatcatgccattgcactccagcctgggcaacagagtgagactgtctcaaaaaaaaaaaaaaaaaccaacaacgacattatgagatttttctttttgcgattttttttttcttttttctgagacagtttcgctattgttgcccaggctggggtgcaatggcgcaatctcagctcaccgcaatctccccctctcaggttcaagcgattctcctgcctcagcctcctgagtagctgggactacaggcatgcaccaccatgcccagctaattttttgtatttttagtaaaaatggggtttctccatgtcggtcaggctggtctcaaactcccgacctaggtgatctcccaaagtgttgggattacaggcgtgagccactacgcccggtccacgattttttttttttttttttttagctcatcagctattgttagtgttagtgtattttatgtgtggtccaagacaattcttcttccattgtggaccagggaagccaaaagattggacacccctgtctagggcaaggattccaaaagtatgttctgtataaaacttgcatagagattccaggaacacttgttcaaatgcaaattcctggtccagatctcaaagatcagtctctgcacgtttggacatttttaacaagcaaccctcatgatttttatgatccttaagtttgacaattctagggccttggtcttcaaaatgacacatgcatacccttgagaacacaccaacattttcccatgggggtaaggatacatgcatagctctatggaaaccaacttaaagatgtccaatttccatatgtgttgtcctaaaatatgtgctctgatgaggcctcttcagatctaccatttctctttacctcccttttcacaacagccatactccctatcctccaaaaaaaaaaaaaaaaaaaaaaaaaaaaagaggctgcctctcaaccatccagtatatcaaggcgtattgccttggtgtaagcagctccagaggcactaaacaaaaggatcaaaaaaaatctaaatgactcctaagacgcaaagagggtagggggcagtagctcaggactgcaatcctagcactttgagaggctgaggcaggagggttgcttgaggctagaagtttgggaccagcctgggcaacatggcaaaatgctgtctgtacaaaaaatacaaaattcagctgggcatggtggtggcacgcgcctatagacccagctacttgggaggcttaggtgggaggattgcttggatctgggaggtcgaggctgcagtgaactgtgattgtgccagtgcactccagcctgggcgacagagcaagaccctgtctcaaaaaacaaaacaaaacaaaacaaaaactgatgcttctgaaggctgtgccagagaagtatgtttgtgtgtttatctgaattaaaaccaagacatgttctgacggaagttaagtctgatttggctaattaaattaagaacagactttgccagtttatatgacaggactttttctataaatttaatcagctaaatctatagtcccagggctttcataaaaatatctttgagccaagcatagtggctcaaggctgtaagcccaacactttgggaggctgaggcgggggaatcacttaaacccaggagttcgagaccagcctgggcaacataacgagacaccgtctacaaattattttaattagctgggagtgatagtgaatgcctgtgagggaagctgaggctggaggatcacttgagcccaggaggtgggccgtgtttgcaccactgcactccagcttggatgacaaagtgagaccgtctctcaaaaaaaaaaaaaaactttaaagcacatatataatatgcaatatgttggatagtatatcctttgtaagtacttaaattttaaaaatttagatttcagattaaagtcttgcaaaagggccagactaggtgcctcatgactataatcccagcaatttggaaggctgaggcgggaggattgtttgagcccaggagttcgagaccagcctgggcaacatagtgagacttcatctccacaaaaaattagccagtgtggttatgctagtctatagtctcagctactcaggaggctgaagtgggaagaccacttatgcccaggaaaccaaggctgcagtgagccatgatcataccactgcactgcacttcagcctgggagacagaacaagacagaccctgtcgccccacacctcccctatacccccggaaaaaaaaaagtgcaaaaaaaaaaaaaactagggtgagagccatgaaatagctgaaggactgtctgaagaggggcagaagggagtgttttggggtgacagaaacattctattgcttttttgggtggttactcagatttctacaactcgttagaaggaaacactttatcatgttaattatacctcaatattgtaaatgtgcatggaagaaatctcttgttttcaagagtttttcttttgggttcacctaactatgtacctgactgctgcataaagtaatccatggcacttaataatttgactaatcagattacttctgttcttcattgttagctccagtatttttcttacagctaccttggattttgatgcctaagaacattctctgacaggttggaaataaaattaaataaaggattgattttcaaataatgtggtaagtgaacggaataaatgcatttttatgttcgtactaccattatgctataaaaaccttaataaccagctgaatctctttcttgcaaatagggcatgaagccccagccttctttagtcttctggcacagtgaaaacaagtgacaagatggcccgtccttccatgaataatgttcccgtctcgtggtcttttctcacataagctacatggcttcaagagattctggcaatcctccatgttttctgtatctgttctctgttcagaaaggttatctaactgttctcccatgcttgagatggtctcttggctttcagaactgtgagccaaatccaagaattccactgagttgcagggatcaaaaagtttggagttttctttctttatatacgcatctttaggtctaacgacaggagccgaaatggttcttcgacaatcagggacatcatttccttcattttccttttcaggtatggcagtgatatcagacgtggagagagaatgggttaactttgaacaatctgaataccaatccttcctcaaggcccaacaacgaaaacagtacctcttgcttggagagttaaatttcttgcattcagtacactgccactcatcctcagaggtaacctctacatcggtatcatcacttaaggacttagagtcctccaggtcatcattttttcccacttcaatcacctgatttgtctgtaaatcagttgagccattacttctaggtgtatagttgcttctcaagtttcctaaaaaccaccaaggcaggccagctacatcccactcctcaaatccaaggtccagcctagatgtttcatcttgggctaaattttcaattaagtcttcatcttctctagaatgtatgcatttatgctctgaggtaggcagtgtggggatatcgtcttctgtagttctttttctggaagtggaactttcctctgcactttgcttcagttggtcttgacttggaatatccatactgtgatcctgtgcgagagcgagagtctgagcagcatctgtagtagcagtggctaaagtgacaagattctttcttagcatatcatagagagggcttgggtctttcacggagaagctctgacgtcccagtagttctcccaaaagatctccaccacaatataccatatgctgctcctgctgatcataaagttgcttcaccattatgtactgacctaaatagtgcatgacctctttaacagtgaacatttcaccttgcgcacctgctgcatgcaaaatcttcaaaagcggcagttttggtcgtacctgattgatttgtccaggagagatcctgcaagcactgtcagatgttgaacactgagcagaggtggaaaatgatgtcattttggtagtgaagaaactgcagtctgttggtaaaacttacggcagctccatgagtcgctcccccgccgagcccgggtggggggaggggtggcagtcacagatcctagggcctcggcagcattttgaaatggcgagtaat

SEQ ID NO: 11084 - RNA, 7210 nt, Homo sapiens
  source 1..7210: mol_type = other RNA
ctgaatagctgggactacaggtgcacgccaccacgaccggctaatttttgtatttttagtagagacagggtttcaccatactggtcagactggtctcgaactcctgagctcaggcaatccacccacctcggcctcccaaagtgctgggattacaggcgtaagccaccgcccctagcctaatatcaatcttcgataaagcatttgccaaattacagcaactgctctgaaagaggaattgctcttctagcattatttgaccctttttaggtatccttgaccctctttaccttaagaaatggagagttccggccgggcgcggtggctcacgcctgtaatcccagtactttgggaggctgaggtgggcagatcacgaggtcaggagatcaagaccatcctggctaagacggtgaaaccccgtctccaataaaaatacaaaaattagccaggcgtggtggcgggcgcctatagtcccagctactagggaggctgaggcaggagaatggggtgaacccgggaggcggaggttgcagtgagccgagatcgcgccactgcactccagccggggcgacagagagagactccgtctaaaaaaaaaaaaaaagaaatggagagttctactaactgtcctgtgctcccagaggggattcaatgaggatcgtaagaaggaaaacaacctgcaggggaagcagcatcttggatttcagataaagtaccaaaaaatattagctatctctttctgcagacatgcctctttctctgttaacactttcagtcattcaaaaggctattggtagaggtgcagcaaatccaagtgtagatttactgtaacagtttatttaactatgctgtattcaccaataacggcattaccaataatggcattagtgcacatcaaaagatctgaaaatgctaatgggacatttcccacaaaaggaaagaaatccaatggctcctataaagggagaatatagcaatggcaagcagaatgaaaatttctgtcaaaagaaagtacttctcaaagcaatcaggaaaaactgttcccaaattaggcctggggagccacattagccactatctcagatactgattattttgtttagccttaggggcctcaatattccccctcatctgctaaacttcaacttgtttactcacaagtctgataaattccagccaagtaaccttaacattccctatggcagtgcaaaattccagacatttgtaaacactgtaaatttcacgtttggtacatgagacagcttaccggttcatctttgattctaaaaacatagctagttcctaatctatggccatttttagcaaaggtagcatcaggatcaaaacatgcttgcacacatgcacactcatgactgggagaaccatcagaactaattgctcgttaggatatagttctgaacaatttaagcagataactgactaaatggaaaacagattcacagtatctaaagccatatatcagaaattcacataattctgaggggaaaaaactcaaatatctagttaacaattgtcttcctttcaaaagcgagtcaagaggtaacattacatagctttgtattatagatcagaagaatattcaccaatatatcaaagacttcaaaaggcagccaacattgcattgaattgacacacacaaaatgttacaaatgaccttgacccttaaaaataaattcttacaaaccaaataataccacacaatgcactacatacatctaactatacataaattataattaaaacacaactgcatatttcaaatgcttggcagtgactcaatcttacattacagaagttagtggcagtgtggaggctggcatggctcaactccaatccattgtacaagcctaggattagaaacccatactattccattggtagactggggaaatggcataccatattaaagatctggtctaagatttttataaagtttgatttaagcattaaataaaaaagcataccaattactgtgaagtacactggaaggagagtgagttaatattcagacagaagaactttttagccgtaatactgaaattcatcgttgttctaatgatttgtcatctctgctctgaacttttcgcccaagataacaatcataaatattaatttgacaactaaaacaagaaatctgatggtaatgtggtgtgatttcattattcatagtctacagcacgttgcagcagaaacaagctccaatgacacagatccttcctcacaatcaagatatcaactcgaacaaggcttacctataactaggtgaccatataatttaacatccaaatgaagaggtttgaaagtgaaaggggacatgcagaaagaaaccaggtgggatgcagaaaaatgggagcaatttggcagtctccagaaaaccagagcacatggtcccaataactacagctaaaaggtaaatgtcagtatttggaagtttccttatagcagtaaactctgaacacttcacatataaactatgccttgctttagtttagtggcagtgagtaaaaaaaatctgtaccgcagtggcaaggaaaaaagaaaatcaaaaacagaccaagaaaatagtttaagctgggcgctgtggctcatgcctgtaatctcagcactttgcgaggctgaggtgggtggatgacctgaggtcaggagttcgagaccagcctgaccaacatggtgaaaccatctctactaaaaatacaaaattagccagacatggtggtgcacacctgtaatcccagctacttgggaggctgaggcaggagaatcatttgaacccgggaggcagaggttgcagtgagccgagatcactccactgcactccagcctgggcgacaagagcaaaactccatctcaagtaaaaaaaaaaaaaaaagaaaagaaaagaaatagtttaaagtttcctacaagtaaagatgaaattcggctcaagcacatatcttaggatcgtctaagtacttagtgctaacagaagcagtgaaaaaccccggtgggcaagcaggaagagtgaagctgagcagcctaagaggattctttcatgggcaatgatgtgtcaaatttaggatcaaatacctataaacataagtaaaatgtttacttcttaagttttattaaaaattacaacttggctgggtgcggtagctcacgcctgtaatcgcaggactttgggaggccgaggtgtgtggatcatgaggtcaggagttcgagaccagcctggccaacacagtgaaacccccatctctactaaaaatacaaaaattagccaggcatggtggtatgtgcctgtagtcccagctatctgggaggctgaggcaggagaatcacctgaacccgggaggcagaggttgcggtgagcagagatcatgccattgcactccagcctgggcaacagagtgagactgtctcaaaaaaaaaaaaaaaaaccaacaacgacattatgagatttttctttttgcgattttttttttcttttttctgagacagtttcgctattgttgcccaggctggggtgcaatggcgcaatctcagctcaccgcaatctccccctctcaggttcaagcgattctcctgcctcagcctcctgagtagctgggactacaggcatgcaccaccatgcccagctaattttttgtatttttagtaaaaatggggtttctccatgtcggtcaggctggtctcaaactcccgacctaggtgatctcccaaagtgttgggattacaggcgtgagccactacgcccggtccacgattttttttttttttttttttagctcatcagctattgttagtgttagtgtattttatgtgtggtccaagacaattcttcttccattgtggaccagggaagccaaaagattggacacccctgtctagggcaaggattccaaaagtatgttctgtataaaacttgcatagagattccaggaacacttgttcaaatgcaaattcctggtccagatctcaaagatcagtctctgcacgtttggacatttttaacaagcaaccctcatgatttttatgatccttaagtttgacaattctagggccttggtcttcaaaatgacacatgcatacccttgagaacacaccaacattttcccatgggggtaaggatacatgcatagctctatggaaaccaacttaaagatgtccaatttccatatgtgttgtcctaaaatatgtgctctgatgaggcctcttcagatctaccatttctctttacctcccttttcacaacagccatactccctatcctccaaaaaaaaaaaaaaaaaaaaaaaaaaaaagaggctgcctctcaaccatccagtatatcaaggcgtattgccttggtgtaagcagctccagaggcactaaacaaaaggatcaaaaaaaatctaaatgactcctaagacgcaaagagggtagggggcagtagctcaggactgcaatcctagcactttgagaggctgaggcaggagggttgcttgaggctagaagtttgggaccagcctgggcaacatggcaaaatgctgtctgtacaaaaaatacaaaattcagctgggcatggtggtggcacgcgcctatagacccagctacttgggaggcttaggtgggaggattgcttggatctgggaggtcgaggctgcagtgaactgtgattgtgccagtgcactccagcctgggcgacagagcaagaccctgtctcaaaaaacaaaacaaaacaaaacaaaaactgatgcttctgaaggctgtgccagagaagtatgtttgtgtgtttatctgaattaaaaccaagacatgttctgacggaagttaagtctgatttggctaattaaattaagaacagactttgccagtttatatgacaggactttttctataaatttaatcagctaaatctatagtcccagggctttcataaaaatatctttgagccaagcatagtggctcaaggctgtaagcccaacactttgggaggctgaggcgggggaatcacttaaacccaggagttcgagaccagcctgggcaacataacgagacaccgtctacaaattattttaattagctgggagtgatagtgaatgcctgtgagggaagctgaggctggaggatcacttgagcccaggaggtgggccgtgtttgcaccactgcactccagcttggatgacaaagtgagaccgtctctcaaaaaaaaaaaaaaactttaaagcacatatataatatgcaatatgttggatagtatatcctttgtaagtacttaaattttaaaaatttagatttcagattaaagtcttgcaaaagggccagactaggtgcctcatgactataatcccagcaatttggaaggctgaggcgggaggattgtttgagcccaggagttcgagaccagcctgggcaacatagtgagacttcatctccacaaaaaattagccagtgtggttatgctagtctatagtctcagctactcaggaggctgaagtgggaagaccacttatgcccaggaaaccaaggctgcagtgagccatgatcataccactgcactgcacttcagcctgggagacagaacaagacagaccctgtcgccccacacctcccctatacccccggaaaaaaaaaagtgcaaaaaaaaaaaaaactagggtgagagccatgaaatagctgaaggactgtctgaagaggggcagaagggagtgttttggggtgacagaaacattctattgcttttttgggtggttactcagatttctacaactcgttagaaggaaacactttatcatgttaattatacctcaatattgtaaatgtgcatggaagaaatctcttgttttcaagagtttttcttttgggttcacctaactatgtacctgactgctgcataaagtaatccatggcacttaataatttgactaatcagattacttctgttcttcattgttagctccagtatttttcttacagctaccttggattttgatgcctaagaacattctctgacaggttggaaataaaattaaataaaggattgattttcaaataatgtggtaagtgaacggaataaatgcatttttatgttcgtactaccattatgctataaaaaccttaataaccagctgaatctctttcttgcaaatagggcatgaagccccagccttctttagtcttctggcacagtgaaaacaagtgacaagatggcccgtccttccatgaataatgttcccgtctcgtggtcttttctcacataagctacatggcttcaagagattctggcaatcctccatgttttctgtatctgttctctgttcagaaaggttatctaactgttctcccatgcttgagatggtctcttggctttcagaactgtgagccaaatccaagaattccactgagttgcagggatcaaaaagtttggagttttctttctttatatacgcatctttaggtctaacgacaggagccgaaatggttcttcgacaatcagggacatcatttccttcattttccttttcaggtatggcagtgatatcagacgtggagagagaatgggttaactttgaacaatctgaataccaatccttcctcaaggcccaacaacgaaaacagtacctcttgcttggagagttaaatttcttgcattcagtacactgccactcatcctcagaggtaacctctacatcggtatcatcacttaaggacttagagtcctccaggtcatcattttttcccacttcaatcacctgtagtagcagtggctaaagtgacaagattctttcttagcatatcatagagagggcttgggtctttcacggagaagctctgacgtcccagtagttctcccaaaagatctccaccacaatataccatatgctgctcctgctgatcataaagttgcttcaccattatgtactgacctaaatagtgcatgacctctttaacagtgaacatttcaccttgcgcacctgctgcatgcaaaatcttcaaaagcggcagttttggtcgtacctgattgatttgtccaggagagatcctgcaagcactgtcagatgttgaacactgagcagaggtggaaaatgatgtcattttggtagtgaagaaactgcagtctgttggtaaaacttacggcagctccatgagtcgctcccccgccgagcccgggtggggggaggggtggcagtcacagatcctagggcctcggcagcattttgaaatggcgagtaat

SEQ ID NO: 11085 - RNA, 7621 nt, Homo sapiens
  source 1..7621: mol_type = other RNA
ctgaatagctgggactacaggtgcacgccaccacgaccggctaatttttgtatttttagtagagacagggtttcaccatactggtcagactggtctcgaactcctgagctcaggcaatccacccacctcggcctcccaaagtgctgggattacaggcgtaagccaccgcccctagcctaatatcaatcttcgataaagcatttgccaaattacagcaactgctctgaaagaggaattgctcttctagcattatttgaccctttttaggtatccttgaccctctttaccttaagaaatggagagttccggccgggcgcggtggctcacgcctgtaatcccagtactttgggaggctgaggtgggcagatcacgaggtcaggagatcaagaccatcctggctaagacggtgaaaccccgtctccaataaaaatacaaaaattagccaggcgtggtggcgggcgcctatagtcccagctactagggaggctgaggcaggagaatggggtgaacccgggaggcggaggttgcagtgagccgagatcgcgccactgcactccagccggggcgacagagagagactccgtctaaaaaaaaaaaaaaagaaatggagagttctactaactgtcctgtgctcccagaggggattcaatgaggatcgtaagaaggaaaacaacctgcaggggaagcagcatcttggatttcagataaagtaccaaaaaatattagctatctctttctgcagacatgcctctttctctgttaacactttcagtcattcaaaaggctattggtagaggtgcagcaaatccaagtgtagatttactgtaacagtttatttaactatgctgtattcaccaataacggcattaccaataatggcattagtgcacatcaaaagatctgaaaatgctaatgggacatttcccacaaaaggaaagaaatccaatggctcctataaagggagaatatagcaatggcaagcagaatgaaaatttctgtcaaaagaaagtacttctcaaagcaatcaggaaaaactgttcccaaattaggcctggggagccacattagccactatctcagatactgattattttgtttagccttaggggcctcaatattccccctcatctgctaaacttcaacttgtttactcacaagtctgataaattccagccaagtaaccttaacattccctatggcagtgcaaaattccagacatttgtaaacactgtaaatttcacgtttggtacatgagacagcttaccggttcatctttgattctaaaaacatagctagttcctaatctatggccatttttagcaaaggtagcatcaggatcaaaacatgcttgcacacatgcacactcatgactgggagaaccatcagaactaattgctcgttaggatatagttctgaacaatttaagcagataactgactaaatggaaaacagattcacagtatctaaagccatatatcagaaattcacataattctgaggggaaaaaactcaaatatctagttaacaattgtcttcctttcaaaagcgagtcaagaggtaacattacatagctttgtattatagatcagaagaatattcaccaatatatcaaagacttcaaaaggcagccaacattgcattgaattgacacacacaaaatgttacaaatgaccttgacccttaaaaataaattcttacaaaccaaataataccacacaatgcactacatacatctaactatacataaattataattaaaacacaactgcatatttcaaatgcttggcagtgactcaatcttacattacagaagttagtggcagtgtggaggctggcatggctcaactccaatccattgtacaagcctaggattagaaacccatactattccattggtagactggggaaatggcataccatattaaagatctggtctaagatttttataaagtttgatttaagcattaaataaaaaagcataccaattactgtgaagtacactggaaggagagtgagttaatattcagacagaagaactttttagccgtaatactgaaattcatcgttgttctaatgatttgtcatctctgctctgaacttttcgcccaagataacaatcataaatattaatttgacaactaaaacaagaaatctgatggtaatgtggtgtgatttcattattcatagtctacagcacgttgcagcagaaacaagctccaatgacacagatccttcctcacaatcaagatatcaactcgaacaaggcttacctataactaggtgaccatataatttaacatccaaatgaagaggtttgaaagtgaaaggggacatgcagaaagaaaccaggtgggatgcagaaaaatgggagcaatttggcagtctccagaaaaccagagcacatggtcccaataactacagctaaaaggtaaatgtcagtatttggaagtttccttatagcagtaaactctgaacacttcacatataaactatgccttgctttagtttagtggcagtgagtaaaaaaaatctgtaccgcagtggcaaggaaaaaagaaaatcaaaaacagaccaagaaaatagtttaagctgggcgctgtggctcatgcctgtaatctcagcactttgcgaggctgaggtgggtggatgacctgaggtcaggagttcgagaccagcctgaccaacatggtgaaaccatctctactaaaaatacaaaattagccagacatggtggtgcacacctgtaatcccagctacttgggaggctgaggcaggagaatcatttgaacccgggaggcagaggttgcagtgagccgagatcactccactgcactccagcctgggcgacaagagcaaaactccatctcaagtaaaaaaaaaaaaaaaagaaaagaaaagaaatagtttaaagtttcctacaagtaaagatgaaattcggctcaagcacatatcttaggatcgtctaagtacttagtgctaacagaagcagtgaaaaaccccggtgggcaagcaggaagagtgaagctgagcagcctaagaggattctttcatgggcaatgatgtgtcaaatttaggatcaaatacctataaacataagtaaaatgtttacttcttaagttttattaaaaattacaacttggctgggtgcggtagctcacgcctgtaatcgcaggactttgggaggccgaggtgtgtggatcatgaggtcaggagttcgagaccagcctggccaacacagtgaaacccccatctctactaaaaatacaaaaattagccaggcatggtggtatgtgcctgtagtcccagctatctgggaggctgaggcaggagaatcacctgaacccgggaggcagaggttgcggtgagcagagatcatgccattgcactccagcctgggcaacagagtgagactgtctcaaaaaaaaaaaaaaaaaccaacaacgacattatgagatttttctttttgcgattttttttttcttttttctgagacagtttcgctattgttgcccaggctggggtgcaatggcgcaatctcagctcaccgcaatctccccctctcaggttcaagcgattctcctgcctcagcctcctgagtagctgggactacaggcatgcaccaccatgcccagctaattttttgtatttttagtaaaaatggggtttctccatgtcggtcaggctggtctcaaactcccgacctaggtgatctcccaaagtgttgggattacaggcgtgagccactacgcccggtccacgattttttttttttttttttttagctcatcagctattgttagtgttagtgtattttatgtgtggtccaagacaattcttcttccattgtggaccagggaagccaaaagattggacacccctgtctagggcaaggattccaaaagtatgttctgtataaaacttgcatagagattccaggaacacttgttcaaatgcaaattcctggtccagatctcaaagatcagtctctgcacgtttggacatttttaacaagcaaccctcatgatttttatgatccttaagtttgacaattctagggccttggtcttcaaaatgacacatgcatacccttgagaacacaccaacattttcccatgggggtaaggatacatgcatagctctatggaaaccaacttaaagatgtccaatttccatatgtgttgtcctaaaatatgtgctctgatgaggcctcttcagatctaccatttctctttacctcccttttcacaacagccatactccctatcctccaaaaaaaaaaaaaaaaaaaaaaaaaaaaagaggctgcctctcaaccatccagtatatcaaggcgtattgccttggtgtaagcagctccagaggcactaaacaaaaggatcaaaaaaaatctaaatgactcctaagacgcaaagagggtagggggcagtagctcaggactgcaatcctagcactttgagaggctgaggcaggagggttgcttgaggctagaagtttgggaccagcctgggcaacatggcaaaatgctgtctgtacaaaaaatacaaaattcagctgggcatggtggtggcacgcgcctatagacccagctacttgggaggcttaggtgggaggattgcttggatctgggaggtcgaggctgcagtgaactgtgattgtgccagtgcactccagcctgggcgacagagcaagaccctgtctcaaaaaacaaaacaaaacaaaacaaaaactgatgcttctgaaggctgtgccagagaagtatgtttgtgtgtttatctgaattaaaaccaagacatgttctgacggaagttaagtctgatttggctaattaaattaagaacagactttgccagtttatatgacaggactttttctataaatttaatcagctaaatctatagtcccagggctttcataaaaatatctttgagccaagcatagtggctcaaggctgtaagcccaacactttgggaggctgaggcgggggaatcacttaaacccaggagttcgagaccagcctgggcaacataacgagacaccgtctacaaattattttaattagctgggagtgatagtgaatgcctgtgagggaagctgaggctggaggatcacttgagcccaggaggtgggccgtgtttgcaccactgcactccagcttggatgacaaagtgagaccgtctctcaaaaaaaaaaaaaaactttaaagcacatatataatatgcaatatgttggatagtatatcctttgtaagtacttaaattttaaaaatttagatttcagattaaagtcttgcaaaagggccagactaggtgcctcatgactataatcccagcaatttggaaggctgaggcgggaggattgtttgagcccaggagttcgagaccagcctgggcaacatagtgagacttcatctccacaaaaaattagccagtgtggttatgctagtctatagtctcagctactcaggaggctgaagtgggaagaccacttatgcccaggaaaccaaggctgcagtgagccatgatcataccactgcactgcacttcagcctgggagacagaacaagacagaccctgtcgccccacacctcccctatacccccggaaaaaaaaaagtgcaaaaaaaaaaaaaactagggtgagagccatgaaatagctgaaggactgtctgaagaggggcagaagggagtgttttggggtgacagaaacattctattgcttttttgggtggttactcagatttctacaactcgttagaaggaaacactttatcatgttaattatacctcaatattgtaaatgtgcatggaagaaatctcttgttttcaagagtttttcttttgggttcacctaactatgtacctgactgctgcataaagtaatccatggcacttaataatttgactaatcagattacttctgttcttcattgttagctccagtatttttcttacagctaccttggattttgatgcctaagaacattctctgacaggttggaaataaaattaaataaaggattgattttcaaataatgtggtaagtgaacggaataaatgcatttttatgttcgtactaccattatgctataaaaaccttaataaccagctgaatctctttcttgcaaatagggcatgaagccccagccttctttagtcttctggcacagtgaaaacaagtgacaagatggcccgtccttccatgaataatgttcccgtctcgtggtcttttctcacataagctacatggcttcaagagattctggcaatcctccatgttttctgtatctgttctctgttcagaaaggttatctaactgttctcccatgcttgagatggtctcttggctttcagaactgtgagccaaatccaagaattccactgagttgcagggatcaaaaagtttggagttttctttctttatatacgcatctttaggtctaacgacaggagccgaaatggttcttcgacaatcagggacatcatttccttcattttccttttcaggtatggcagtgatatcagacgtggagagagaatgggttaactttgaacaatctgaataccaatccttcctcaaggcccaacaacgaaaacagtacctcttgcttggagagttaaatttcttgcattcagtacactgccactcatcctcagaggtaacctctacatcggtatcatcacttaaggacttagagtcctccaggtcatcattttttcccacttcaatcacctttttgtcacttactttccctacttcttcacttgtttgttcagtatcagcagcttcaacttttattccaacacctaactgctctgatactgactcattcaaaaaccacaagtcatctgtagtatctgaaacaatggcagtacccacatcctgatttgtctgtaaatcagttgagccattacttctaggtgtatagttgcttctcaagtttcctaaaaaccaccaaggcaggccagctacatcccactcctcaaatccaaggtccagcctagatgtttcatcttgggctaaattttcaattaagtcttcatcttctctagaatgtatgcatttatgctctgaggtaggcagtgtggggatatcgtcttctgtagttctttttctggaagtggaactttcctctgcactttgctgtagtagcagtggctaaagtgacaagattctttcttagcatatcatagagagggcttgggtctttcacggagaagctctgacgtcccagtagttctcccaaaagatctccaccacaatataccatatgctgctcctgctgatcataaagttgcttcaccattatgtactgacctaaatagtgcatgacctctttaacagtgaacatttcaccttgcgcacctgctgcatgcaaaatcttcaaaagcggcagttttggtcgtacctgattgatttgtccaggagagatcctgcaagcactgtcagatgttgaacactgagcagaggtggaaaatgatgtcattttggtagtgaagaaactgcagtctgttggtaaaacttacggcagctccatgagtcgctcccccgccgagcccgggtggggggaggggtggcagtcacagatcctagggcctcggcagcattttgaaatggcgagtaat

SEQ ID NO: 11086 - RNA, 7395 nt, Homo sapiens
  source 1..7395: mol_type = other RNA
ctgaatagctgggactacaggtgcacgccaccacgaccggctaatttttgtatttttagtagagacagggtttcaccatactggtcagactggtctcgaactcctgagctcaggcaatccacccacctcggcctcccaaagtgctgggattacaggcgtaagccaccgcccctagcctaatatcaatcttcgataaagcatttgccaaattacagcaactgctctgaaagaggaattgctcttctagcattatttgaccctttttaggtatccttgaccctctttaccttaagaaatggagagttccggccgggcgcggtggctcacgcctgtaatcccagtactttgggaggctgaggtgggcagatcacgaggtcaggagatcaagaccatcctggctaagacggtgaaaccccgtctccaataaaaatacaaaaattagccaggcgtggtggcgggcgcctatagtcccagctactagggaggctgaggcaggagaatggggtgaacccgggaggcggaggttgcagtgagccgagatcgcgccactgcactccagccggggcgacagagagagactccgtctaaaaaaaaaaaaaaagaaatggagagttctactaactgtcctgtgctcccagaggggattcaatgaggatcgtaagaaggaaaacaacctgcaggggaagcagcatcttggatttcagataaagtaccaaaaaatattagctatctctttctgcagacatgcctctttctctgttaacactttcagtcattcaaaaggctattggtagaggtgcagcaaatccaagtgtagatttactgtaacagtttatttaactatgctgtattcaccaataacggcattaccaataatggcattagtgcacatcaaaagatctgaaaatgctaatgggacatttcccacaaaaggaaagaaatccaatggctcctataaagggagaatatagcaatggcaagcagaatgaaaatttctgtcaaaagaaagtacttctcaaagcaatcaggaaaaactgttcccaaattaggcctggggagccacattagccactatctcagatactgattattttgtttagccttaggggcctcaatattccccctcatctgctaaacttcaacttgtttactcacaagtctgataaattccagccaagtaaccttaacattccctatggcagtgcaaaattccagacatttgtaaacactgtaaatttcacgtttggtacatgagacagcttaccggttcatctttgattctaaaaacatagctagttcctaatctatggccatttttagcaaaggtagcatcaggatcaaaacatgcttgcacacatgcacactcatgactgggagaaccatcagaactaattgctcgttaggatatagttctgaacaatttaagcagataactgactaaatggaaaacagattcacagtatctaaagccatatatcagaaattcacataattctgaggggaaaaaactcaaatatctagttaacaattgtcttcctttcaaaagcgagtcaagaggtaacattacatagctttgtattatagatcagaagaatattcaccaatatatcaaagacttcaaaaggcagccaacattgcattgaattgacacacacaaaatgttacaaatgaccttgacccttaaaaataaattcttacaaaccaaataataccacacaatgcactacatacatctaactatacataaattataattaaaacacaactgcatatttcaaatgcttggcagtgactcaatcttacattacagaagttagtggcagtgtggaggctggcatggctcaactccaatccattgtacaagcctaggattagaaacccatactattccattggtagactggggaaatggcataccatattaaagatctggtctaagatttttataaagtttgatttaagcattaaataaaaaagcataccaattactgtgaagtacactggaaggagagtgagttaatattcagacagaagaactttttagccgtaatactgaaattcatcgttgttctaatgatttgtcatctctgctctgaacttttcgcccaagataacaatcataaatattaatttgacaactaaaacaagaaatctgatggtaatgtggtgtgatttcattattcatagtctacagcacgttgcagcagaaacaagctccaatgacacagatccttcctcacaatcaagatatcaactcgaacaaggcttacctataactaggtgaccatataatttaacatccaaatgaagaggtttgaaagtgaaaggggacatgcagaaagaaaccaggtgggatgcagaaaaatgggagcaatttggcagtctccagaaaaccagagcacatggtcccaataactacagctaaaaggtaaatgtcagtatttggaagtttccttatagcagtaaactctgaacacttcacatataaactatgccttgctttagtttagtggcagtgagtaaaaaaaatctgtaccgcagtggcaaggaaaaaagaaaatcaaaaacagaccaagaaaatagtttaagctgggcgctgtggctcatgcctgtaatctcagcactttgcgaggctgaggtgggtggatgacctgaggtcaggagttcgagaccagcctgaccaacatggtgaaaccatctctactaaaaatacaaaattagccagacatggtggtgcacacctgtaatcccagctacttgggaggctgaggcaggagaatcatttgaacccgggaggcagaggttgcagtgagccgagatcactccactgcactccagcctgggcgacaagagcaaaactccatctcaagtaaaaaaaaaaaaaaaagaaaagaaaagaaatagtttaaagtttcctacaagtaaagatgaaattcggctcaagcacatatcttaggatcgtctaagtacttagtgctaacagaagcagtgaaaaaccccggtgggcaagcaggaagagtgaagctgagcagcctaagaggattctttcatgggcaatgatgtgtcaaatttaggatcaaatacctataaacataagtaaaatgtttacttcttaagttttattaaaaattacaacttggctgggtgcggtagctcacgcctgtaatcgcaggactttgggaggccgaggtgtgtggatcatgaggtcaggagttcgagaccagcctggccaacacagtgaaacccccatctctactaaaaatacaaaaattagccaggcatggtggtatgtgcctgtagtcccagctatctgggaggctgaggcaggagaatcacctgaacccgggaggcagaggttgcggtgagcagagatcatgccattgcactccagcctgggcaacagagtgagactgtctcaaaaaaaaaaaaaaaaaccaacaacgacattatgagatttttctttttgcgattttttttttcttttttctgagacagtttcgctattgttgcccaggctggggtgcaatggcgcaatctcagctcaccgcaatctccccctctcaggttcaagcgattctcctgcctcagcctcctgagtagctgggactacaggcatgcaccaccatgcccagctaattttttgtatttttagtaaaaatggggtttctccatgtcggtcaggctggtctcaaactcccgacctaggtgatctcccaaagtgttgggattacaggcgtgagccactacgcccggtccacgattttttttttttttttttttagctcatcagctattgttagtgttagtgtattttatgtgtggtccaagacaattcttcttccattgtggaccagggaagccaaaagattggacacccctgtctagggcaaggattccaaaagtatgttctgtataaaacttgcatagagattccaggaacacttgttcaaatgcaaattcctggtccagatctcaaagatcagtctctgcacgtttggacatttttaacaagcaaccctcatgatttttatgatccttaagtttgacaattctagggccttggtcttcaaaatgacacatgcatacccttgagaacacaccaacattttcccatgggggtaaggatacatgcatagctctatggaaaccaacttaaagatgtccaatttccatatgtgttgtcctaaaatatgtgctctgatgaggcctcttcagatctaccatttctctttacctcccttttcacaacagccatactccctatcctccaaaaaaaaaaaaaaaaaaaaaaaaaaaaagaggctgcctctcaaccatccagtatatcaaggcgtattgccttggtgtaagcagctccagaggcactaaacaaaaggatcaaaaaaaatctaaatgactcctaagacgcaaagagggtagggggcagtagctcaggactgcaatcctagcactttgagaggctgaggcaggagggttgcttgaggctagaagtttgggaccagcctgggcaacatggcaaaatgctgtctgtacaaaaaatacaaaattcagctgggcatggtggtggcacgcgcctatagacccagctacttgggaggcttaggtgggaggattgcttggatctgggaggtcgaggctgcagtgaactgtgattgtgccagtgcactccagcctgggcgacagagcaagaccctgtctcaaaaaacaaaacaaaacaaaacaaaaactgatgcttctgaaggctgtgccagagaagtatgtttgtgtgtttatctgaattaaaaccaagacatgttctgacggaagttaagtctgatttggctaattaaattaagaacagactttgccagtttatatgacaggactttttctataaatttaatcagctaaatctatagtcccagggctttcataaaaatatctttgagccaagcatagtggctcaaggctgtaagcccaacactttgggaggctgaggcgggggaatcacttaaacccaggagttcgagaccagcctgggcaacataacgagacaccgtctacaaattattttaattagctgggagtgatagtgaatgcctgtgagggaagctgaggctggaggatcacttgagcccaggaggtgggccgtgtttgcaccactgcactccagcttggatgacaaagtgagaccgtctctcaaaaaaaaaaaaaaactttaaagcacatatataatatgcaatatgttggatagtatatcctttgtaagtacttaaattttaaaaatttagatttcagattaaagtcttgcaaaagggccagactaggtgcctcatgactataatcccagcaatttggaaggctgaggcgggaggattgtttgagcccaggagttcgagaccagcctgggcaacatagtgagacttcatctccacaaaaaattagccagtgtggttatgctagtctatagtctcagctactcaggaggctgaagtgggaagaccacttatgcccaggaaaccaaggctgcagtgagccatgatcataccactgcactgcacttcagcctgggagacagaacaagacagaccctgtcgccccacacctcccctatacccccggaaaaaaaaaagtgcaaaaaaaaaaaaaactagggtgagagccatgaaatagctgaaggactgtctgaagaggggcagaagggagtgttttggggtgacagaaacattctattgcttttttgggtggttactcagatttctacaactcgttagaaggaaacactttatcatgttaattatacctcaatattgtaaatgtgcatggaagaaatctcttgttttcaagagtttttcttttgggttcacctaactatgtacctgactgctgcataaagtaatccatggcacttaataatttgactaatcagattacttctgttcttcattgttagctccagtatttttcttacagctaccttggattttgatgcctaagaacattctctgacaggttggaaataaaattaaataaaggattgattttcaaataatgtggtaagtgaacggaataaatgcatttttatgttcgtactaccattatgctataaaaaccttaataaccagctgaatctctttcttgcaaatagggcatgaagccccagccttctttagtcttctggcacagtgaaaacaagtgacaagatggcccgtccttccatgaataatgttcccgtctcgtggtcttttctcacataagctacatggcttcaagagattctggcaatcctccatgttttctgtatctgttctctgttcagaaaggttatctaactgttctcccatgcttgagatggtctcttggctttcagaactgtgagccaaatccaagaattccactgagttgcagggatcaaaaagtttggagttttctttctttatatacgcatctttaggtctaacgacaggagccgaaatggttcttcgacaatcagggacatcatttccttcattttccttttcaggtatggcagtgatatcagacgtggagagagaatgggttaactttgaacaatctgaataccaatccttcctcaaggcccaacaacgaaaacagtacctcttgcttggagagttaaatttcttgcattcagtacactgccactcatcctcagaggtaacctctacatcggtatcatcacttaaggacttagagtcctccaggtcatcattttttcccacttcaatcacctttttgtcacttactttccctacttcttcacttgtttgttcagtatcagcagcttcaacttttattccaacacctaactgctctgatactgactcattcaaaaaccacaagtcatctgtagtatctgaaacaatggcagtacccacatcctgatttgtctgtaaatcagttgagccattacttctaggtgtatagttgcttctcaagtttcctaaaaaccaccaaggcaggccagctacatcccactcctcaaatccaaggtccagcctagatgtttcatcttgggctaaattttcaattaagtcttcatcttctctagaatgtatgcatttatgctctgaggtaggcagtgtggggatatcgtcttctgtagttctttttctggaagtggaactttcctctgcactttgcttcagttggtcttgacttggaatatccatactgtgatcctgattgatttgtccaggagagatcctgcaagcactgtcagatgttgaacactgagcagaggtggaaaatgatgtcattttggtagtgaagaaactgcagtctgttggtaaaacttacggcagctccatgagtcgctcccccgccgagcccgggtggggggaggggtggcagtcacagatcctagggcctcggcagcattttgaaatggcgagtaat

SEQ ID NO: 11087 - RNA, 7689 nt, Homo sapiens
  source 1..7689: mol_type = other RNA
ctgaatagctgggactacaggtgcacgccaccacgaccggctaatttttgtatttttagtagagacagggtttcaccatactggtcagactggtctcgaactcctgagctcaggcaatccacccacctcggcctcccaaagtgctgggattacaggcgtaagccaccgcccctagcctaatatcaatcttcgataaagcatttgccaaattacagcaactgctctgaaagaggaattgctcttctagcattatttgaccctttttaggtatccttgaccctctttaccttaagaaatggagagttccggccgggcgcggtggctcacgcctgtaatcccagtactttgggaggctgaggtgggcagatcacgaggtcaggagatcaagaccatcctggctaagacggtgaaaccccgtctccaataaaaatacaaaaattagccaggcgtggtggcgggcgcctatagtcccagctactagggaggctgaggcaggagaatggggtgaacccgggaggcggaggttgcagtgagccgagatcgcgccactgcactccagccggggcgacagagagagactccgtctaaaaaaaaaaaaaaagaaatggagagttctactaactgtcctgtgctcccagaggggattcaatgaggatcgtaagaaggaaaacaacctgcaggggaagcagcatcttggatttcagataaagtaccaaaaaatattagctatctctttctgcagacatgcctctttctctgttaacactttcagtcattcaaaaggctattggtagaggtgcagcaaatccaagtgtagatttactgtaacagtttatttaactatgctgtattcaccaataacggcattaccaataatggcattagtgcacatcaaaagatctgaaaatgctaatgggacatttcccacaaaaggaaagaaatccaatggctcctataaagggagaatatagcaatggcaagcagaatgaaaatttctgtcaaaagaaagtacttctcaaagcaatcaggaaaaactgttcccaaattaggcctggggagccacattagccactatctcagatactgattattttgtttagccttaggggcctcaatattccccctcatctgctaaacttcaacttgtttactcacaagtctgataaattccagccaagtaaccttaacattccctatggcagtgcaaaattccagacatttgtaaacactgtaaatttcacgtttggtacatgagacagcttaccggttcatctttgattctaaaaacatagctagttcctaatctatggccatttttagcaaaggtagcatcaggatcaaaacatgcttgcacacatgcacactcatgactgggagaaccatcagaactaattgctcgttaggatatagttctgaacaatttaagcagataactgactaaatggaaaacagattcacagtatctaaagccatatatcagaaattcacataattctgaggggaaaaaactcaaatatctagttaacaattgtcttcctttcaaaagcgagtcaagaggtaacattacatagctttgtattatagatcagaagaatattcaccaatatatcaaagacttcaaaaggcagccaacattgcattgaattgacacacacaaaatgttacaaatgaccttgacccttaaaaataaattcttacaaaccaaataataccacacaatgcactacatacatctaactatacataaattataattaaaacacaactgcatatttcaaatgcttggcagtgactcaatcttacattacagaagttagtggcagtgtggaggctggcatggctcaactccaatccattgtacaagcctaggattagaaacccatactattccattggtagactggggaaatggcataccatattaaagatctggtctaagatttttataaagtttgatttaagcattaaataaaaaagcataccaattactgtgaagtacactggaaggagagtgagttaatattcagacagaagaactttttagccgtaatactgaaattcatcgttgttctaatgatttgtcatctctgctctgaacttttcgcccaagataacaatcataaatattaatttgacaactaaaacaagaaatctgatggtaatgtggtgtgatttcattattcatagtctacagcacgttgcagcagaaacaagctccaatgacacagatccttcctcacaatcaagatatcaactcgaacaaggcttacctataactaggtgaccatataatttaacatccaaatgaagaggtttgaaagtgaaaggggacatgcagaaagaaaccaggtgggatgcagaaaaatgggagcaatttggcagtctccagaaaaccagagcacatggtcccaataactacagctaaaaggtaaatgtcagtatttggaagtttccttatagcagtaaactctgaacacttcacatataaactatgccttgctttagtttagtggcagtgagtaaaaaaaatctgtaccgcagtggcaaggaaaaaagaaaatcaaaaacagaccaagaaaatagtttaagctgggcgctgtggctcatgcctgtaatctcagcactttgcgaggctgaggtgggtggatgacctgaggtcaggagttcgagaccagcctgaccaacatggtgaaaccatctctactaaaaatacaaaattagccagacatggtggtgcacacctgtaatcccagctacttgggaggctgaggcaggagaatcatttgaacccgggaggcagaggttgcagtgagccgagatcactccactgcactccagcctgggcgacaagagcaaaactccatctcaagtaaaaaaaaaaaaaaaagaaaagaaaagaaatagtttaaagtttcctacaagtaaagatgaaattcggctcaagcacatatcttaggatcgtctaagtacttagtgctaacagaagcagtgaaaaaccccggtgggcaagcaggaagagtgaagctgagcagcctaagaggattctttcatgggcaatgatgtgtcaaatttaggatcaaatacctataaacataagtaaaatgtttacttcttaagttttattaaaaattacaacttggctgggtgcggtagctcacgcctgtaatcgcaggactttgggaggccgaggtgtgtggatcatgaggtcaggagttcgagaccagcctggccaacacagtgaaacccccatctctactaaaaatacaaaaattagccaggcatggtggtatgtgcctgtagtcccagctatctgggaggctgaggcaggagaatcacctgaacccgggaggcagaggttgcggtgagcagagatcatgccattgcactccagcctgggcaacagagtgagactgtctcaaaaaaaaaaaaaaaaaccaacaacgacattatgagatttttctttttgcgattttttttttcttttttctgagacagtttcgctattgttgcccaggctggggtgcaatggcgcaatctcagctcaccgcaatctccccctctcaggttcaagcgattctcctgcctcagcctcctgagtagctgggactacaggcatgcaccaccatgcccagctaattttttgtatttttagtaaaaatggggtttctccatgtcggtcaggctggtctcaaactcccgacctaggtgatctcccaaagtgttgggattacaggcgtgagccactacgcccggtccacgattttttttttttttttttttagctcatcagctattgttagtgttagtgtattttatgtgtggtccaagacaattcttcttccattgtggaccagggaagccaaaagattggacacccctgtctagggcaaggattccaaaagtatgttctgtataaaacttgcatagagattccaggaacacttgttcaaatgcaaattcctggtccagatctcaaagatcagtctctgcacgtttggacatttttaacaagcaaccctcatgatttttatgatccttaagtttgacaattctagggccttggtcttcaaaatgacacatgcatacccttgagaacacaccaacattttcccatgggggtaaggatacatgcatagctctatggaaaccaacttaaagatgtccaatttccatatgtgttgtcctaaaatatgtgctctgatgaggcctcttcagatctaccatttctctttacctcccttttcacaacagccatactccctatcctccaaaaaaaaaaaaaaaaaaaaaaaaaaaaagaggctgcctctcaaccatccagtatatcaaggcgtattgccttggtgtaagcagctccagaggcactaaacaaaaggatcaaaaaaaatctaaatgactcctaagacgcaaagagggtagggggcagtagctcaggactgcaatcctagcactttgagaggctgaggcaggagggttgcttgaggctagaagtttgggaccagcctgggcaacatggcaaaatgctgtctgtacaaaaaatacaaaattcagctgggcatggtggtggcacgcgcctatagacccagctacttgggaggcttaggtgggaggattgcttggatctgggaggtcgaggctgcagtgaactgtgattgtgccagtgcactccagcctgggcgacagagcaagaccctgtctcaaaaaacaaaacaaaacaaaacaaaaactgatgcttctgaaggctgtgccagagaagtatgtttgtgtgtttatctgaattaaaaccaagacatgttctgacggaagttaagtctgatttggctaattaaattaagaacagactttgccagtttatatgacaggactttttctataaatttaatcagctaaatctatagtcccagggctttcataaaaatatctttgagccaagcatagtggctcaaggctgtaagcccaacactttgggaggctgaggcgggggaatcacttaaacccaggagttcgagaccagcctgggcaacataacgagacaccgtctacaaattattttaattagctgggagtgatagtgaatgcctgtgagggaagctgaggctggaggatcacttgagcccaggaggtgggccgtgtttgcaccactgcactccagcttggatgacaaagtgagaccgtctctcaaaaaaaaaaaaaaactttaaagcacatatataatatgcaatatgttggatagtatatcctttgtaagtacttaaattttaaaaatttagatttcagattaaagtcttgcaaaagggccagactaggtgcctcatgactataatcccagcaatttggaaggctgaggcgggaggattgtttgagcccaggagttcgagaccagcctgggcaacatagtgagacttcatctccacaaaaaattagccagtgtggttatgctagtctatagtctcagctactcaggaggctgaagtgggaagaccacttatgcccaggaaaccaaggctgcagtgagccatgatcataccactgcactgcacttcagcctgggagacagaacaagacagaccctgtcgccccacacctcccctatacccccggaaaaaaaaaagtgcaaaaaaaaaaaaaactagggtgagagccatgaaatagctgaaggactgtctgaagaggggcagaagggagtgttttggggtgacagaaacattctattgcttttttgggtggttactcagatttctacaactcgttagaaggaaacactttatcatgttaattatacctcaatattgtaaatgtgcatggaagaaatctcttgttttcaagagtttttcttttgggttcacctaactatgtacctgactgctgcataaagtaatccatggcacttaataatttgactaatcagattacttctgttcttcattgttagctccagtatttttcttacagctaccttggattttgatgcctaagaacattctctgacaggttggaaataaaattaaataaaggattgattttcaaataatgtggtaagtgaacggaataaatgcatttttatgttcgtactaccattatgctataaaaaccttaataaccagctgaatctctttcttgcaaatagggcatgaagccccagccttctttagtcttctggcacagtgaaaacaagtgacaagatggcccgtccttccatgaataatgttcccgtctcgtggtcttttctcacataagctacatggcttcaagagattctggcaatcctccatgttttctgtatctgttctctgttcagaaaggttatctaactgttctcccatgcttgagatggtctcttggctttcagaactgtgagccaaatccaagaattccactgagttgcagggatcaaaaagtttggagttttctttctttatatacgcatctttaggtctaacgacaggagccgaaatggttcttcgacaatcagggacatcatttccttcattttccttttcaggtatggcagtgatatcagacgtggagagagaatgggttaactttgaacaatctgaataccaatccttcctcaaggcccaacaacgaaaacagtacctcttgcttggagagttaaatttcttgcattcagtacactgccactcatcctcagaggtaacctctacatcggtatcatcacttaaggacttagagtcctccaggtcatcattttttcccacttcaatcacctttttgtcacttactttccctacttcttcacttgtttgttcagtatcagcagcttcaacttttattccaacacctaactgctctgatactgactcattcaaaaaccacaagtcatctgtagtatctgaaacaatggcagtacccacatcctgatttgtctgtaaatcagttgagccattacttctaggtgtatagttgcttctcaagtttcctaaaaaccaccaaggcaggccagctacatcccactcctcaaatccaaggtccagcctagatgtttcatcttgggctaaattttcaattaagtcttcatcttctctagaatgtatgcatttatgctctgaggtaggcagtgtggggatatcgtcttctgtagttctttttctggaagtggaactttcctctgcactttgcttcagttggtcttgacttggaatatccatactgtgatcctgtgcgagagcgagagtctgagcagcatctgtagtagcagtggctaaagtgacaagattctttcttagcatatcatagagagggcttgggtctttcacggagaagctctgacgtcccagtagttctcccaaaagatctccaccacaatataccatatgctgctcctgctgatcataaagttgcttcaccattatgtactgacctaaatagtgcatgacctctttaacagtgaacatttcaccttgcgcacctgctgcatgcaaaatcttcaaaagcggcagttttggtcgtacctgattgatttgtccaggagagatcctgcaagcactgtcagatgttgaacactgagcagaggtggaaaatgatgtcattttggtagtgaagaaactgcagtctgttggtaaaacttacggcagctccatgagtcgctcccccgccgagcccgggtggggggaggggtggcagtcacagatcctagggcctcggcagcattttgaaatggcgagtaat

SEQ ID NO: 11088 - RNA, 3846 nt, Homo sapiens
  source 1..3846: mol_type = other RNA
ctgaatagctgggactacaggtgcacgccaccacgcccagctaatttttgtatttttaatagagacggggtttcaccatgtttgccaggctggtcttgaactcctggcctcaagtgatccagctgccttagcctcccaaagtgttgggattacaggcatgagccaccatgcccggccttttcttcttctatttttatttttttaaatacaatccacggtcctggactagatttcaggacttttcaagagaagctggaaatccattttgcctgagaaatgtgttgttgttgctatgccaaattaaatgcacacatgactggatttgttgtttctgcatgttgtaatagttctgagcatgagttcgggagtctggggtttgaattttggcggtaccactcatccattctgcataattgagggtcccagtttcctcgtctctaaaatggaattctacctcataaggttgtgtgggtttttttttttttgagatagagtctcgctgtcgcccaggcagcagtgcagtgctgtgatcttggctcactgcaacctccgccttccaggttcaaacaattctcttttctcagcctcctgaagagctgggactacaggtgcacaccactacacctggctaatttttctatttttagtagagatggggtttcaccatattggtcaggctggtctcgaactcctgaccccaggtgacccacctgccttggcctcccaaagtgctgagattacaggcgtgagccaccatgcccggccctcaagatttttatgaggaccacatgaaatgctgaaagcacttagtagtatgtccaggagcagggtcttgctctgtcatctagacttgaatgcagcgagtggcatcgtcatagctcactgcaggctcaatctctcagcctcaagcaatccttgcccctcagcctcctaagtagctgggactacacgtccagctaatttttgtatttttgtaaagatggggcctcactatgttgccttggctggtcttgaactcctagtttcaagttatcctctcaccttggcctcccgaagtgttgggattataggcgtgagccactgcaactggccaggacagtgattgattgattgattgattggtttgagacagagtctcactctgtcgtccaggatggagtgcagtggcacgatctcagctcactgtaacctccacctcccgggttcaagcaattctgctgcctcagcctctcgagtaggtgggattacaggcacattccaccatgcccggctaatttttgtatttttaggagagacagggtttcaccatactggccattgctggtctcgaactcttgacttcatgatccgcccgcctaggcctcccaaagtgctgggattgacagtggcatttaaatagagaccttttagaaaagtgggaaagtagaaaaataaataataaatacataaatagagacctgtaaatgatgaacagtgaacttggtggagaagtgagatgggcatggggaggatagccctcaagcagagggaacagggtagaaatcaatcatgcaacaccaaattcaagcagtgaggatagaggggacagccaatcctctagggagggctaaggatttcctgactgataaagcctgagcggcaaagaagcctcctatccagccttgggcaagtctctgccaagctgggacttcacactacactggccagccattgacttccctgatagaaaaaccacaaccaacaagtcctcgctggggctggtctgccaaacacagaagacagagggaaggggagggggctgtcttggggtcagaagtgagcaggttttccaggggagaaggaagattgagaagaggggtatggctgctggctcacacctataatcccaacacttagggaggccaaggcgggaggcacacttgtggccaggagttcgagaccagcctgggcaacatagcgagacttcgtctgaacaaaaaaaaattatagtttaaaaattagctgggtgtagtggcgcgtgcctgaagtcccaggtattcacaaggctgagggaggaggatcgcttaagcccaggaggtcgaggctgcagcaaactatgatcctgcaactgcactccaacccaagtgacagagcaagaccttaaaacacacacaaaaaaaaccaaaaaacggcagaaagatgagaagccgttccatttgcataggcagttgaagtgtctaggcagaggcctccaaggctgactggatatcaggcaggggatgaggctggacagcctgcaatgcctccaactccaggttgcggaaatcgtgtttgtagtacctcagtcgaatggagattgagcgccccctgggagcagtgctcggtaacagacgctggaggaccccgatgaggaggggcgggggtcggttcaatctgggaggagcctgcgggtcagttttcttctcacaggagcgaactctgtccggcatcatggattcctgggctcccagaacggctgggctggaagggaccttagaaagggatctaccaccgcgtgccccgtgccagagttgggcactttggtgacaagaacattggcttgtttaacactcacaactgtgcttcgaggtggggatcattatccccattgtccccattttgcagatgagaaaaagcaaggtttggtggcttcccggggcggggcggggattcgctgtgactccaggtccttttccccggagcccgcacgtcttgtaagacactgattcccggaggtctgaggagcaggaatcgagtgggaggtgcccaggctttctagggaacaagagtgtgaatgcactctcgacgagaaccacgcccccctgttcgacaagactgattcctgctgccttcctttaagggccctcccctgaaacgcgaagtcctcgccccatggagaggcggacattctttattcccggatcgcccgacgtttttctcccccacccgcactgatccccactggtgacataaatccttcccctccactcgcgagtgaaagcttgggactacatttcccgccaggctgttcagaagccggtggcggagagaggagaaaagagtctttccgtttccgtcgcctcgcaatttggcgtgtccgccgggattcacatttcaacagcgacgtcctttctctgttggactcggcaaggaactacatttcccagcaggcaccggcgcagaggtcgaggggcgaggtcgccatctttttcgtagtcctctccctcatttccgcagggaagaggccagacgcctggactacacatcccatgtcgcagtcgccccggccctgcagccgccatctttgccggtggccccgccccatccccttccattgtctcgacttgagatgatagacgggagccgggagactgcaactcccgtcaggccgtgcgccactggtgggggggatttcgagaccacaggcgggcgaggtgcccaaggtggtggaaagcggagaccgggagaggctaggtagcctgccatctttacggtagtctcctcgtcctcctggttccgccattcttaaggaacactggaaggctataaaactactaatcccatcgcacctcgtaagatcgactactagtcaggtgtatgtccctcttccgccatcttgcttgtagtcctctttccttttcacctttccattgttcctgacgagtagaaatggcagcgggaaggcagcagatggactgcgactcccgtcaggtaccacacacgcggagggttgtggacaggagggcgtgtgagtgcctgggaaggaggtcgggtcgggggagaaggccatcttgtttgtagtcatcgttccctctccttctcgatgtt

SEQ ID NO: 11089 - RNA, 13792 nt, Homo sapiens
  source 1..13792: mol_type = other RNA
ctgaatagctgggactacaggtgcacgccaccacgcccagctaatttttgtatttttagtagagacagggtttcaccatattgaccaggctgctctcaaactcctgaccttatgatctgcccacctcagcctcccaaagtgttaggattacaggcgtgagccaccgcgcctggcctctttcatctattttaacttgttttcttttttcttttttttgagatagggtcttgctctgtcacccaggctggagtacagtggcatgctcatggatcactacaaccttgacctcctgggctcaagtgatcctctcaccatagcctcctgagtagctgggactacagatgcacatgaccatgaccagctaacttgttttttctgtagagacatgactttgccatgttgcccaggctggtctgaaactcctggactcaagcaatctgcccctttgcctcccaaagtgctaagactacaggcatgggccgtcatacccagccaactttttaaatataatgtaaggtaagtgtccaacttcattcttttgcacgtgactatccacttgtcccagcaccatttgttgaaaagactgttctttccccactgaatggacttggcacctttactgaaaatcagttgactacagatgtttgcatttatttctggaatcaccattttttaaaaaaatacaatgatctatgtctacccttgtgccagtaacacacttcttaattactattgttttgtaattcaaaatgaagaaatgtgggtttttctactttattctttttcaggatttctttggctattctgggtcccttgaaatttcatataactcttagcatcagcttgtcaatttctgcaaagatgtcagcagagattctgacagggattatgctgaatctgcagacaagtttgaggaatattgtcatcttaacagcattaactcttctgatccatgaacatggcatgtttttccatttatttaggtcttctttaattactttctgcaatgttttgtagttttcagagtgtaagttttgcactttttgttaaatatgttattaagcaccttattctttttgatgctattatgaatattcttaatttcatttttgattattcattgcaagtgtgtagaaatacgatttttttttttttgagatggagtctcgctttgtcacccaggctggagtgcggtggcacaatcttggctcactgcaagctccgcctcccaggttcatgccattctcctgcctcagcctcccaagtagctgggactacaggcacccgccaccacgcctggctaattttttgtatttttagtggagacagggtttcaccgtgttagccaggatggtcttgatctcctgacctcatgatccacctgcctcggcctcccaaagtgctgggattacaggcgtgagccaccatgcccggcccaactgatttttaaatactgatgttgtatcctcccatcttgctgaactcacttattagtttcaatagtttttttttttttttttggtggattccctagaatcttctacatacaagatcatgtcatttgtgaacagtctttcttcttcctttccaacctttattttcttcttgcataattgcaatggcttagaccctccagtacaatgttaaatagaagtgtgataatgggcatccttgtcttatttctaatctcagtgggaaagcattcagtttttcaccattaagtataaagaaagctgtagatttttcatagatgttctttatcaggttaaggtagtttccttccgttcctcgtttttcaaacatttttatgatgaaagggtgttggatttattcaaatgcagctatttttgcatcagtagagatgacttttttattatattgatataatgtattacattgattttcacatgttaagccaatcttatatccctgggataaatcctacttggtgatggtgcataattatttttatatgttgctggatttggtttgcagcatttagttgaggatttttgcaggtatttcataagacatattggtctgcagttttcttgtaatatctttgagcagttttgttatcagggcaatactgggaagtactccctcctatttcttgaaagagtttgagaataattgctataatttatttgattgtttggtagaacacagtggtaaaactgtctgtgcctggactattctttgtgggcaattttctgattcctggtttaatctgttcactagttataggtctattcagattgcccatttctgtaaggttggtagtagtgtctactctttcatatcagatcctagtaatttgagtattgcctttttattggtcaacctagtgaaatatttgtcatatttattgatcttttcaaattaccagtttctagtaatattttctctattgtttttctattctttcattaatttctactctaattttattatttccttccttctgcttgctttaggtttagtttgttcttctttcttcagtgacttaaggtggaagaaaggttattgctttatttcttccttaatacaggcatttacacctataaatttcctctaagcacttttttagctgcatccgtacagtttacttgtgtcttaattttcattagcctcaaagtgctgattaccttcttgttttcttctttggtctattggtcatttagtagtgtgttgttcaatttcctaattgtgagttcttcaaatgttcccattttttatttctaatttaatcctgtgattatgttcacaaaatgcactttgcattatttctatccttttaaacgtattgaagtttcatggtctagcataaggcctatcctgaagaatgttctatgagcatttgataatgtatatgctgtagcgcttgggtgaagtgttctatagatgtctgttagggctagttggtttacagcgttggtcaagttttctatttcattgttaaccttgtgtctagttttgtccattactgaaaataggttatggagtctccaattattattgtgaccattttcttcttccatttctgtcagtttttgctttctgtgttttgatactgttaagttcatacatatgtttacaactgttatatctttttgatgggttaacctttttatcattataaaatgtctctatctctaggagcatttttgtcttaaagtctactttgtctgacactagtatagccagtccagctttcttatggcaattgtttgcactatttctttttgtatccttttaatctatctgtgtctttgagcctaaagtgtgttatctatgggagcatagataacatagagttggaatgtatttttaatccaatctgatagtctctgcctgattaaattcattaacatttattattgataagttgaatacacattactttttgttttctagtatccattgtgttcttttcattctcttttaatattgccttttgcatcgagtattttctaaggtagtattttaatttgattaatgatttttcaactatatttctggagttattttattagtggttgctctagtgtttaccatatacatcttatcagaatctgttagaattacacaagcttaactccaataatatatagaagctttactcttatatagctatattccctttccccctttttgtgatattttaggtatacatatggtatctattaatgttacaaatccaacacattgttataattattactttaccatctgccatcatttaattagtctactacagctttgctcccagccacctcctttgtgctgttttgacaaatgttacatatatgacatttctgtatgttatagaccaatacatcatatacgtattatttgatacagttgcattttaatcagttaagaggagaaaaatatgcatttatgtgacttttataattatataattgcttttactggtgctcttctcttgctttcagcctaaagaacttcatttaatacttcttattaggcaggttggttaacaacaatttttctgtttttgtttatctgggaaagtatttcacttatatttttgaataatacatttgctggatataggattcttggttgacagtttttttttcttcaagcactttgactgttatacctgccttctggcctccattatttcttttgagaagtcaagtattaattttgttctctaagtgatgtatctttttttcactcactactttcaaggttttctcatctttgatttcagcatttttgactatgatgtgtctgtgaatccctctgcatttatcatgctggaagttcactaagcttcctagatgtttttcaatcaatttggagagttttcagtcattgtatctttaaatatttcctttttcttctgctcttcttgtactcccattacatgcatacttaatggtgcacataatggtgcttcacatttctctgaggttttgctcatttttcattttttttctctctgttctttggaaagcatatctctcttattctatctgccagttggctgacaatttcttctgccagttcaaatctactattgaacccctttagtgcattttttccttattatagtttttaacttcatgaatttagctcttgccacttgaagctggaggggataagaaatgctggcatcttgcccctccctgtgaggtaccatacctctggacagggagctgagggagacggagctctgttttcttggctgcacccactgaaatgggagggagggagtgagtgtgttgtggctgaaatgtctgactcactgttcttaccaagatttggattttcttgaataagcgttactttattctacatgcttttaggacaatttccagtggcattaagtgtttgtgtctctctgtatgagaggaaggtgtttattttttgttacaattttcactagttatagctaattcctaggacagtgggtccacagggcccttcacattgccattctggaagtgaaaatctaaaagatatttcaatgttagaaaatttaactgtgtactttactacaccaagaaaagctatacaattatatcaatatataccagaaaagactttgaggacaatcattctaccatttgtgataatcaattatgataccacaatgataaaaacagtgggttactaagcaaagttagataaatggaccaatttaacagaatgcagagccaagaaacatttccgtacattatatgtaaattggtaaaggtggccttatacatcaggaggaaaataataaactattttttaaaggtgctagggaaactagctatccatatgggattaataattcataagaatgtattcatgaccctagctagggaatggttcttaaataaacaaaaaaaaatggaaagactgaatttactatattttaaaacttccgtatgataaacatcacaaaatagatatgtgaatatgctaattctccatatttttatgtaagttaaaagactcacaaccaaaactaaaaatctataaaacacctaggaataagcctattatgaaatgtgcaagacatttatgaagaaagttattaaaatttcatccaagaatataaaagactttaataaaatgaggcctatcataacactaatcagaaacattatattaattataaagaggtctattattctcaaattaatgtgtaaacaaatgcaatcctagtcaaaagaacaccacaattttactggaatttaataaactaattcttgattcagctggaacagaaaacacccaagtataagacactgaagagggggagaaaggaaaaggaacttgcccatgaatggcaaaacacaatgcaaagcaccaaatgacagcgtgaggagtgtggttggtagaaccaacacctggatccacaggacagaaatagacaacttagcatgtgatgagttgaaagctgacattttaaactggtggagaaaagaatatttgttgatcattggaataactgcctttttgtttttgtttaggggagcaatcctaaaagataaacaacccacaggaaaactaggccaacataacactaataggcaatgtacggtagagatctacaaatggccaataaacatggaaatgtttgattttgtacgtaatcagggaaattcaagtgaaaacaaggtactttcaatcacgagactggttaaaacaaaacaaaacaacctatcgatattgataccacttactgttggcaagggtttggagaaatgggtccttttatggagggtgaattgatgcaagcaattctgctacatccactgacatttaaaatctacatcattaatccaacaattctgtgcaggcagagctatacttacaggaatagaaatgtcttgcatataatattaaatgaaaagttagttgcaaaataaggatggtataaggccattaatataaattacatatttaaagcaaactaattgctataatagacttcaaaagacagtagcttaagcaagtcagtattttattttactcttaaataacaggtcaaaggagagcagttcaagactggcaggccaacttctccttcctcaacacatcacttccatctcttgagatgccaggtcactactgaagctcccattggcctcccagccagcaagaaaggggaatgtcaaggagagtgcataccctgcttctttaaagggccaattgggaagtttaaaacttagtcatatggccacaattaactataagagaggctgagaagtagtcttaagctgagcagccagacgtccaggtaaaactcaaaaattttattagtaaaggaagaatgggaaaatgacattatagcagcagtctgtgtcatgtgattctctaaatgcatggagaatacacaccaaacctagggctgtacttagctgtggaacaggtgcaagatggtgtgggggtggggaggcagactattgcttgaacatttttaatggtgatagtattaacatttaattttttgacaaaattttaaaatcctttatttgtgctgataaagcatgttaaatacattaaatctatttacactgtacaaagcttttaaagttctaaaaatcagatttttatctaaatgaataaatttctctgtattgttaaaaccattctacttaactgcattgttctccaagtccctccagccaggaggcacggtaacaatgtgtcagatctccacactgagacaccaccttcccaagatcatggtacatcagcagcagaactgagacaaaaactggaacaaggaccaccttgctcctactgcattatagcttttgatagtatttgctacttgaagaggaggctataccttgtctagctcaatacagtttatgtttcagacactataagtatgatacccaaatgcttcatgagtgaacaaggtcagcagatcaccctgagaacaaggaagacacaatttccttataggctaatgattataaaaatagaaattaagagctccccagaaacaaaccacttagtcaaaaaggaaggagttttgactttcttctaagccaagtactcaagtttaagacttattggcctatttaaaaattctttctatgacttctaaacaatgatggcaaagtgacaaaaataatgtaatcatcttcttccctcattatatataaaccaaactaaaaacaaaagaaatgaacaagctataatccaaaaaaaactagaaaatcctgacaggaatcatatagaacatctctaagaaaaggattcttggcttaagcaaaatattagagcagagaaagcaaaactcatgtcctctcatgcagtccggcaaggcccccctgcccagaaccctcctctctgagtcacatggatgagcagacagaagatctggacacagctatccatgttaagcatgagagagatgtaaagaaatagcagggtaggagggcaggcatactacagaaaaatgagagagaggaaaagagcatgccagagaatacaaatccaagaaacaaactgcactaagacagctaagaagaaatttcaggaatacgatgaatttcggaaaacaacacttcaaagatgagatgataaaatcatcctgagaaggaaacaagaaaaacatgggtaagaaaataaactgaggatcaaagcaacaccatcacagaaccacaaacacataaacagtagtgagatacaaacagccttggctggaatccaaaccgcagaaacaagaaagcccgtcgcaaggaatgcaaaggcaggcgcaagacgaaggcaactggagagaagacagcctgccagcctgcagacaagagaggcctggagtggtgtcacttcatggtaacaacggctgggtctgctgtgggctgcagtgatgtttgtgtgcatgcatgtgtgtggtttttatgtacctacttttggctttaatttgattttttttaatgataacacattttgtgactgtaggagagaaaaagatgccctctgcttaaaggaaagccagggtaaactgaataccctacagctttccacaaatacatgtcttatcatttattaccatactatttcatgctttactaataaaaatactcaccaatttaccagtaccttgaaaagaggatctttccaagaaaattaatataattatcaaacaacaaataacaaacctgacctttgtgggtggcaaatggtaaatataaatgtttaaagtttaagcatcaaaataatgctgttatcagatattgatgaacttattgaacaggtctgactgaatgtaagacctgtttttagcaccaataaaaaaaaatattgagatttctgttctgcaaacttctaactgtgctccctgacagcatcttttgggtaaaggaacaaatgtgctccaaggagtaactgttaggtacctgatttacaatataattagattgccaaaaaaaaaaaaatcaatccaagtattttctcctttagctagcattattaaaacttttaactttcagagaagagtttcttcttccttaaagttttaattctgaggtagacatcatgcaaacaaacatcaagtgcagccaacttccattgacaaacatgattattaataataaattaataatcagaaatgcccgttagaaaaagggacttgaaagtttaggaagcaatgttgtttagcagtattctggcttgagtttccaaattccttcaccaccagaagttctatggaaagtgcacagatttctcaatagttctcggaagacacaagactgtgatgcagataacttggattcaaactcctgcagtatctccctggtgctggcctggccatcagtgtgggcctggaaagcgatgaagtttctcatctccaccagaaggtcatcgtgttctgtggtgggcagcagggcagaagcttcctgcaggtgcccgctttcactttctaaacgctctggcagaatcaggtggtttctagctctcattttagccaagagtgaggaggaagcgaggggcccggatgaagagtctgcatcttctgctcttccactaaaatgctcagggacattatcttttccctcctttttcatgatgccatcctggcacttctctgttggagatgttgatgaaggatgctgcacagagaagttagaattccttttcttaccaaatctactcttttttcctgctggtgcaccagaaatccccctgtggccagtccaggtgggaacaccagacactgctcccagacaccgctgacgagagagcctcagtgctttcagggcatcctgggccactcggttggcttctgcctccaccagtacataatctgggctggctccatccatgatggcatcgtgcttcatgacactgtgcacgccaactgattttttgaaaagcttttccaaaacataatcgtcattgctctgttccttggcctcactcttgttttcactgtcttgcttctggtaacgccttttcttcaccaggtgtggaattcgagttccttcaaacttggcgtctctgcaatgcttagagttcttaggcttttgctttggtctcagatgtttctccagggtctcttcttctgccacactatgatgttttgtttttgacttgtgcttataaaaattattttccatttgtttattctcccaaaaagcttctgtttgagcctggctgggtctttctcttttgtaagaaagacctaacttttcatcaatgctttcatcaccagatggcatagaagttttgcctgttcctgaagaatttgaacattccccatttccactaatcactgacaactcttctggtccagatactgcatttgtctcttctccaagcctatcattgctagttacattactactcatgtgagggtcatctttcaaaggatcacttcgattagaagttactgcatttacttcagctcctttagcctcagatttctcttcagatgatgtggcatcatttacagatatgttagaagcagggaacttcttgcgttttggaacatcatggtctgctccaaaggctggttgaatccttctttttagatggcatttgggtgtctgaacatctgatccagttcctgcaaaaattgcacttgtttcagtgctctgggatgcatcaggactagtcagagtaaatagctcatagagatcattggatttgaaaaaccgcctttgttttgggtcttttagcactctatttgtcaaaaactgcttgaagatttgtcggtggtagatcttttcttcaatggtgcccgcagtcaggagcctgtacacagtcacttgcttcttctggcctattctccatgctcgctcccgggcctgcgtgtccgtgcttgggttccagtctgggtcatagatgacaactctgtttgcccccgtcaggttgacacctaagccgcccacccgcgtggtcagaagaaacacaaatatggatgtgtcctcattgtatctcgtaatcagtggctgtcttgaagctattgtagtggtaccatccatcttgagataggtatacttttgggctctaaggaatacttcaagtatgtccagcatctgccttgactgagaaaacagcaatactcgctgaccctgcttgtgccatattttcaacaaagactcaacaacaatcattttcccagaacgtttccagtacccaaactgatcttcttctagttcatcatcaggaagacctttgagattcttgggacctccagaaaagagatcagggtggttgcaaatttttcttagggctataagtccggagaaaatctgcatctctccattgagaatcctgtaaacttctttggaatcaacgaaattttggtagactttatgctgctcatctgtaagacggcaaaataagacctgttcatttttatctggcaaagaaaggctcatcttgacatctgacttcattctccgcagtaggtatggatttatggtatctcgtaagacacatgcacacttgtaagcagttttgacctgtactggggaagcatttgaatatccccccatggtgatggggacggagaactgctccataaacacaggcaacgtgcctaactttcccgggaagatgaagtcaaagagcgaccacagctctcggaggttattttgcatcggtgagccagacagaatgatccgatgaggggtgcgaaactgtttgcaagcaagggtgacagcagcatttggatttcgaattttgtgtccttcgtccaagatcacatagtgccagtcatacctgctaatgtcatcctgcatcaatcgaatgtaggagtaagatgtgatcaaaattccatgacaatgagcaacatctcgaattagtttctcctttttgtgggtataggaaccggtttcatgtagaattgccactctgaacggaggccaccacgtgtgaaattccttcacccactgatgcatcactgttgttggacagacaattacagttggacccaacccctcaaacctgtaatttgaaccacgagtcctgatcttgctgtagctcagacctgccaagaaggcaattatctggatggtcttgcccaatcccatttcatctcccagaattcctcctgcctgctggcagtgcaattcccacagccacctaacacctgtctgctggtacttaaaaagctttttgaacagaaaacctggcactttaaaaccttcgtcaaattcagcatcactttcctcagaatcgtcctccagcttcagacgtttctctttgtcctgcagtctcagtttattccatctccttaaccgctgcttataataatcttcatctccatcatctcggtatcttcccactttccgacctcctcctcctccttctcctacagaagcagcttcagcttcttccccagaacttgggaaaaagtcatcatcaatctcctgcactggcactttcttctgccgtttcccgcccttgggcagaggcttcagctcatagtcagtaccatctccagacaggtccgcctctgccccctccacctcgtcatcttcctcctcttcctcctcctctgtggggaaatactcagactcttcaccctcagagtctccctctgcctctggcctcatgtctgactcccaaggtctccttgcctttggcaatcccactttcccctggaactgcaaagccctcttctggagtttcttgatgtgctttttcaaacgctcctcttttttggacagaactctggctttcttgtttggtttgtttttattttgcactggggctggaggcgtgactggggctggagcttttctagctgctcttttattacaaccttgcttcttcctttcaaaagacagttttgcttgatctgccaaatacttttcgaagcctgatgcttcattaagcatgatttttctgggctttttctcctgtttctgagggatctgggtaccaaaaggtgtcatctggccagtgcggatgagctcttcccaggcagtctcctggacaggcatgagcatgctgccaagactggatggccccggctctgcatcctcctccagactggcgtgatctagttcaattttcacctctgctcctccaaggatggcctggagatgcttttgttttgcagtgatcttttttagctgttgttccttattatacttctgtcgttttacagaatctagtttcctgttgatgtctctgctggtggcagcttgagggctaagctgttcaataattttattgatttgccttagggatgtcgtacatgacgtgaggtcatccaggaccgaccgatactccttctccacgtcaacgagctgggaggcacggctggcctcatggatggcattgtccacctgctgaagcactccctgttccagcacgtcctggtcatagacgtccacacccaaaccctgcagctcaagggcctgggcgctaggctctactgcctggatctgatgtcggtcgatgtgcagcagggctggccctctcctcggagctgctgatgcgcaccccacagcagaggtggacagcccgtcacccacagaacgaaaggagaggtactcctccacctccccatcaccaccactttcttgcttgattgccatttcttcattattactgacaggttgactctgtaaacagtcttgctcctgagtttgacttgagtgggggattccctcatttggcattctctacagaccagggccgcgcgagcgcccacaaggaaacagagacgctaccgccgccagccgccttggaacccagctcgacgggccgtggcgcctgcgccctcagctcaaccatagacaccgcccccaacagcgactccgacttctgctggtgcggggaggcccgtggc

SEQ ID NO: 11090 - RNA, 1949 nt, Homo sapiens
  source 1..1949: mol_type = other RNA
ctgaatagctgggactacaggtgcacgccaccacgcccagctaatttttgtatttttagtagagacggggtttcaccatgttggccaggatggtctccatctcttgacctcgtgatccacctgcctcggcctcccaaagtgctgggattacaggcgtgagccaccacgcccagcccatcctttctcctcttaaattttctttgctgaccagtatctcttgatgtggaacgttctttcattagtggtaatactgtcaatcaggtctttggaagatattttgggttttgtttgctgaaccattatgcttattttacaaattaacttttctgaactttattgtggtagaatttacataacaatttaccattttgaccatttttaagttcaaaggaactaagtacattcacattgctatgcaactatgactaccatctagctccagaaccttttcatcttctcaaactgaaattctgtacccattaaacaataagctcccagccgggcacagtggctcgcgcctgtaatcccagcactttgggaggctgaggtgggcggattacctggagtcaggagttcgagaccagcctggccaacatgatggccatctctactaagaatacaaaaattagctggttgtggtgatgaatgcctgtaatcccagctacgtgggaggctgaggcatgagaatcacttgaacctgggaggcagacgttgcagtgagctgggattgcaccactgcactccagcctaggcaacagaaggagactcccgtctcaaaaaaaaaaaaacaaaacaaaaacaagaaccaataagctcccattccttctgccttccagcccttggcaaccaccattccactttaaatttgattattctaggagttcataaaagtggggtaacacagtatttgtcattttgtgactgacttatttcacctatcataaagtcttcaagattcatccaagatgtaatatatatcagaagtttcctcctttttaaggctgagtaatattccattgtgtgtatatgtcacatttcttttaaccattcatcccttgatggacacttggattgcttccaccttctggctattgtgaatgctgctgctgtgaacatagatgtacaaattatctgtccaagttcctgcttttacttcttttgggtatatacccggaagtggaattgctggatataattttaatttttgaggaatctccatactcagatgatcttatttccttatttttcaagtgtgtgggtctatgtgtggttttggcagggaagcgagtctctgttattcccacatactccccatgactgttaagtgctgtgttagaagcatatggtttgatgagaattctaggagagacaaatgtttcaaaggatctctgtattttcaccggcaataactaataaatcatctggcttcgctgttccccaccatgtagttgtggcattttgggaattagtacactcaggagagaagctgtgtttaggatgaagtgagttggatcatacttcgtatagaaacttgccagaaaatatagaattattggagaaattgtgaaaaacttccgtgaagatgtaaactgtactccatagtccagttgttcccaatgagttaggagccttgctttaccctggtcaggagtttcgaaaggtgttcctttcactgcatgcaaaaatacgtacatccccagattatgtataatatttgttaaagtccaagcaacaggaacactgaagaagggaatgctgagtaagacaatatgaagcaagccaactcccaatgcatatgtcagccacataccccggctgttcatgacacgggtatttggattcacttcactgtgggcaactccaacgttcatgtttgctccgccgccccactccgggccgccggctcgcagcaggaccagcccggctgctacggccgcggatacacgccc

SEQ ID NO: 11091 - RNA, 1843 nt, Homo sapiens
  source 1..1843: mol_type = other RNA
ctgaatagctgggactacaggtgcacgccaccacgcccagctaatttttgtatttttagtagagacggggtttcaccatgttggccaggatggtctccatctcttgacctcgtgatccacctgcctcggcctcccaaagtgctgggattacaggcgtgagccaccacgcccagcccatcctttctcctcttaaattttctttgctgaccagtatctcttgatgtggaacgttctttcattagtggtaatactgtcaatcaggtctttggaagatattttgggttttgtttgctgaaccattatgcttattttacaaattaacttttctgaactttattgtggtagaatttacataacaatttaccattttgaccatttttaagttcaaaggaactaagtacattcacattgctatgcaactatgactaccatctagctccagaaccttttcatcttctcaaactgaaattctgtacccattaaacaataagctcccagccgggcacagtggctcgcgcctgtaatcccagcactttgggaggctgaggtgggcggattacctggagtcaggagttcgagaccagcctggccaacatgatggccatctctactaagaatacaaaaattagctggttgtggtgatgaatgcctgtaatcccagctacgtgggaggctgaggcatgagaatcacttgaacctgggaggcagacgttgcagtgagctgggattgcaccactgcactccagcctaggcaacagaaggagactcccgtctcaaaaaaaaaaaaacaaaacaaaaacaagaaccaataagctcccattccttctgccttccagcccttggcaaccaccattccactttaaatttgattattctaggagttcataaaagtggggtaacacagtatttgtcattttgtgactgacttatttcacctatcataaagtcttcaagattcatccaagatgtaatatatatcagaagtttcctcctttttaaggctgagtaatattccattgtgtgtatatgtcacatttcttttaaccattcatcccttgatggacacttggattgcttccaccttctggctattgtgaatgctgctgctgtgaacatagatgtacaaattatctgtccaagttcctgcttttacttcttttgggtatatacccggaagtggaattgctggatataattttaatttttgaggaatctccatactcagatgatcttatttccttatttttcaagtgtgtgggtctatgtgtggttttggcagggaagcgagtctctgttattcccacatactccccatgactgttaagtgctgtgttagaagcatatggtttgatgagaattctaggagagacaaatgtttcaaaggatctctgtattttcaccggcaataactaataaatcatctggcttcgctgttccccagaattattggagaaattgtgaaaaacttccgtgaagatgtaaactgtactccatagtccagttgttcccaatgagttaggagccttgctttaccctggtcaggagtttcgaaaggtgttcctttcactgcatgcaaaaatacgtacatccccagattatgtataatatttgttaaagtccaagcaacaggaacactgaagaagggaatgctgagtaagacaatatgaagcaagccaactcccaatgcatatgtcagccacataccccggctgttcatgacacgggtatttggattcacttcactgtgggcaactccaacgttcatgtttgctccgccgccccactccgggccgccggctcgcagcaggaccagcccggctgctacggccgcggatacacgccc

SEQ ID NO: 11092 - RNA, 1887 nt, Homo sapiens
  source 1..1887: mol_type = other RNA
ctgaatagctgggactacaggtgcacgccaccacgcccagctaatttttgtatttttagtagagacggggtttcaccatgttggccaggatggtctccatctcttgacctcgtgatccacctgcctcggcctcccaaagtgctgggattacaggcgtgagccaccacgcccagcccatcctttctcctcttaaattttctttgctgaccagtatctcttgatgtggaacgttctttcattagtggtaatactgtcaatcaggtctttggaagatattttgggttttgtttgctgaaccattatgcttattttacaaattaacttttctgaactttattgtggtagaatttacataacaatttaccattttgaccatttttaagttcaaaggaactaagtacattcacattgctatgcaactatgactaccatctagctccagaaccttttcatcttctcaaactgaaattctgtacccattaaacaataagctcccagccgggcacagtggctcgcgcctgtaatcccagcactttgggaggctgaggtgggcggattacctggagtcaggagttcgagaccagcctggccaacatgatggccatctctactaagaatacaaaaattagctggttgtggtgatgaatgcctgtaatcccagctacgtgggaggctgaggcatgagaatcacttgaacctgggaggcagacgttgcagtgagctgggattgcaccactgcactccagcctaggcaacagaaggagactcccgtctcaaaaaaaaaaaaacaaaacaaaaacaagaaccaataagctcccattccttctgccttccagcccttggcaaccaccattccactttaaatttgattattctaggagttcataaaagtggggtaacacagtatttgtcattttgtgactgacttatttcacctatcataaagtcttcaagattcatccaagatgtaatatatatcagaagtttcctcctttttaaggctgagtaatattccattgtgtgtatatgtcacatttcttttaaccattcatcccttgatggacacttggattgcttccaccttctggctattgtgaatgctgctgctgtgaacatagatgtacaaattatctgtccaagttcctgcttttacttcttttgggtatatacccggaagtggaattgctggatataattttaatttttgaggaatctccatactcagatgatcttatttccttatttttcaagtgtgtgggtctatgtgtggttttggcagggaagcgagtctctgttattcccacatactccccatgactgttaagtgctgtgttagaagcatatggtttgatgagaattctaggagagacaaatgtttcaaaggatctctgtattttcaccggcaataactaataaatcatctggcttcgctgttccccagaattattggagaaattgtgaaaaacttccgtgaagatgtaaactgtactccatagtccagttgttcccaatgagttaggagccttgctttaccctggtcaggagtttcgaaaggtgttcctttcactgcatgcaaaaatacgtacatccccagattatgtataatatttgttaaagtccaagcaacaggaacactgaagaagggaatgctgagtaagacaatatgaagcaagccaactcccaatgcatatgtcagccacataccccggctgttcatgacacgggtatttggattcacttcactgtgggcaactccaacgttcatgtttgctcgtgaagaggctgttggctctgccctcgccggtgcctccgaagacggcgacccgcagcggcccctcaggggagtcccccctgctagaccgacagcccgagcgctctgggccagag

SEQ ID NO: 11093 - RNA, 2038 nt, Homo sapiens
  source 1..2038: mol_type = other RNA
ctgaatagctgggactacaggtgcacgccaccacgcccagctaatttttgtatttttagtagagacggggtttcaccatgttggccaggatggtctccatctcttgacctcgtgatccacctgcctcggcctcccaaagtgctgggattacaggcgtgagccaccacgcccagcccatcctttctcctcttaaattttctttgctgaccagtatctcttgatgtggaacgttctttcattagtggtaatactgtcaatcaggtctttggaagatattttgggttttgtttgctgaaccattatgcttattttacaaattaacttttctgaactttattgtggtagaatttacataacaatttaccattttgaccatttttaagttcaaaggaactaagtacattcacattgctatgcaactatgactaccatctagctccagaaccttttcatcttctcaaactgaaattctgtacccattaaacaataagctcccagccgggcacagtggctcgcgcctgtaatcccagcactttgggaggctgaggtgggcggattacctggagtcaggagttcgagaccagcctggccaacatgatggccatctctactaagaatacaaaaattagctggttgtggtgatgaatgcctgtaatcccagctacgtgggaggctgaggcatgagaatcacttgaacctgggaggcagacgttgcagtgagctgggattgcaccactgcactccagcctaggcaacagaaggagactcccgtctcaaaaaaaaaaaaacaaaacaaaaacaagaaccaataagctcccattccttctgccttccagcccttggcaaccaccattccactttaaatttgattattctaggagttcataaaagtggggtaacacagtatttgtcattttgtgactgacttatttcacctatcataaagtcttcaagattcatccaagatgtaatatatatcagaagtttcctcctttttaaggctgagtaatattccattgtgtgtatatgtcacatttcttttaaccattcatcccttgatggacacttggattgcttccaccttctggctattgtgaatgctgctgctgtgaacatagatgtacaaattatctgtccaagttcctgcttttacttcttttgggtatatacccggaagtggaattgctggatataattttaatttttgaggaatctccatactcagatgatcttatttccttatttttcaagtgtgtgggtctatgtgtggttttggcagggaagcgagtctctgttattcccacatactccccatgactgttaagtgctgtgttagaagcatatggtttgatgagaattctaggagagacaaatgtttcaaaggatctctgtattttcaccggcaataactaataaatcatctggcttcgctgttcccccactccttccttataagaaattcagtagctgtaaaattttttttcagtttcaaaacatttcaatacttattaattccaaagatccgaacaccatgtagttgtggcattttgggaattagtacactcaggagagaagctgtgtttaggatgaagtgagttggatcatacttcgtatagaaacttgccagaaaatatagaattattggagaaattgtgaaaaacttccgtgaagatgtaaactgtactccatagtccagttgttcccaatgagttaggagccttgctttaccctggtcaggagtttcgaaaggtgttcctttcactgcatgcaaaaatacgtacatccccagattatgtataatatttgttaaagtccaagcaacaggaacactgaagaagggaatgctgagtaagacaatatgaagcaagccaactcccaatgcatatgtcagccacataccccggctgttcatgacacgggtatttggattcacttcactgtgggcaactccaacgttcatgtttgctccgccgccccactccgggccgccggctcgcagcaggaccagcccggctgctacggccgcggatacacgccc

SEQ ID NO: 11094 - RNA, 1972 nt, Homo sapiens
  source 1..1972: mol_type = other RNA
ctgaatagctgggactacaggtgcacgccaccacgcccagctaatttttgtatttttagtagagacggggtttcaccatgttggccaggatggtctccatctcttgacctcgtgatccacctgcctcggcctcccaaagtgctgggattacaggcgtgagccaccacgcccagcccatcctttctcctcttaaattttctttgctgaccagtatctcttgatgtggaacgttctttcattagtggtaatactgtcaatcaggtctttggaagatattttgggttttgtttgctgaaccattatgcttattttacaaattaacttttctgaactttattgtggtagaatttacataacaatttaccattttgaccatttttaagttcaaaggaactaagtacattcacattgctatgcaactatgactaccatctagctccagaaccttttcatcttctcaaactgaaattctgtacccattaaacaataagctcccagccgggcacagtggctcgcgcctgtaatcccagcactttgggaggctgaggtgggcggattacctggagtcaggagttcgagaccagcctggccaacatgatggccatctctactaagaatacaaaaattagctggttgtggtgatgaatgcctgtaatcccagctacgtgggaggctgaggcatgagaatcacttgaacctgggaggcagacgttgcagtgagctgggattgcaccactgcactccagcctaggcaacagaaggagactcccgtctcaaaaaaaaaaaaacaaaacaaaaacaagaaccaataagctcccattccttctgccttccagcccttggcaaccaccattccactttaaatttgattattctaggagttcataaaagtggggtaacacagtatttgtcattttgtgactgacttatttcacctatcataaagtcttcaagattcatccaagatgtaatatatatcagaagtttcctcctttttaaggctgagtaatattccattgtgtgtatatgtcacatttcttttaaccattcatcccttgatggacacttggattgcttccaccttctggctattgtgaatgctgctgctgtgaacatagatgtacaaattatctgtccaagttcctgcttttacttcttttgggtatatacccggaagtggaattgctggatataattttaatttttgaggaatctccatactcagatgatcttatttccttatttttcaagtgtgtgggtctatgtgtggttttggcagggaagcgagtctctgttattcccacatactccccatgactgttaagtgctgtgttagaagcatatggtttgatgagaattctaggagagacaaatgtttcaaaggatctctgtattttcaccggcaataactaataaatcatctggcttcgctgttccccttattaattccaaagatccgaacaccatgtagttgtggcattttgggaattagtacactcaggagagaagctgtgtttaggatgaagtgagttggatcatacttcgtatagaaacttgccagaaaatatagaattattggagaaattgtgaaaaacttccgtgaagatgtaaactgtactccatagtccagttgttcccaatgagttaggagccttgctttaccctggtcaggagtttcgaaaggtgttcctttcactgcatgcaaaaatacgtacatccccagattatgtataatatttgttaaagtccaagcaacaggaacactgaagaagggaatgctgagtaagacaatatgaagcaagccaactcccaatgcatatgtcagccacataccccggctgttcatgacacgggtatttggattcacttcactgtgggcaactccaacgttcatgtttgctccgccgccccactccgggccgccggctcgcagcaggaccagcccggctgctacggccgcggatacacgccc

SEQ ID NO: 11095 - RNA, 2082 nt, Homo sapiens
  source 1..2082: mol_type = other RNA
ctgaatagctgggactacaggtgcacgccaccacgcccagctaatttttgtatttttagtagagacggggtttcaccatgttggccaggatggtctccatctcttgacctcgtgatccacctgcctcggcctcccaaagtgctgggattacaggcgtgagccaccacgcccagcccatcctttctcctcttaaattttctttgctgaccagtatctcttgatgtggaacgttctttcattagtggtaatactgtcaatcaggtctttggaagatattttgggttttgtttgctgaaccattatgcttattttacaaattaacttttctgaactttattgtggtagaatttacataacaatttaccattttgaccatttttaagttcaaaggaactaagtacattcacattgctatgcaactatgactaccatctagctccagaaccttttcatcttctcaaactgaaattctgtacccattaaacaataagctcccagccgggcacagtggctcgcgcctgtaatcccagcactttgggaggctgaggtgggcggattacctggagtcaggagttcgagaccagcctggccaacatgatggccatctctactaagaatacaaaaattagctggttgtggtgatgaatgcctgtaatcccagctacgtgggaggctgaggcatgagaatcacttgaacctgggaggcagacgttgcagtgagctgggattgcaccactgcactccagcctaggcaacagaaggagactcccgtctcaaaaaaaaaaaaacaaaacaaaaacaagaaccaataagctcccattccttctgccttccagcccttggcaaccaccattccactttaaatttgattattctaggagttcataaaagtggggtaacacagtatttgtcattttgtgactgacttatttcacctatcataaagtcttcaagattcatccaagatgtaatatatatcagaagtttcctcctttttaaggctgagtaatattccattgtgtgtatatgtcacatttcttttaaccattcatcccttgatggacacttggattgcttccaccttctggctattgtgaatgctgctgctgtgaacatagatgtacaaattatctgtccaagttcctgcttttacttcttttgggtatatacccggaagtggaattgctggatataattttaatttttgaggaatctccatactcagatgatcttatttccttatttttcaagtgtgtgggtctatgtgtggttttggcagggaagcgagtctctgttattcccacatactccccatgactgttaagtgctgtgttagaagcatatggtttgatgagaattctaggagagacaaatgtttcaaaggatctctgtattttcaccggcaataactaataaatcatctggcttcgctgttccccttattaattccaaagatccgaacaccatgtagttgtggcattttgggaattagtacactcaggagagaagctgtgtttaggatgaagtgagttggatcatacttcgtatagaaacttgccagaaaatatagaattattggagaaattgtgaaaaacttccgtgaagatgtaaactgtactccatagtccagttgttcccaatgagttaggagccttgctttaccctggtcaggagtttcgaaaggtgttcctttcactgcatgcaaaaatacgtacatccccagattatgtataatatttgttaaagtccaagcaacaggaacactgaagaagggaatgctgagtaagacaatatgaagcaagccaactcccaatgcatatgtcagccacataccccggctgttcatgacacgggtatttggattcacttcactgtgggcaactccaacgttcatgtttgctcgagccagtgtgtcaagtagtcagactcttatatttgacttaatgtatccataaagaatggtcagagttcagatcacttctttctgaatactcaatgtggaaggtacatgccgccgccccactccgggccgccggctcgcagcaggaccagcccggctgctacggccgcggatacacgccc

SEQ ID NO: 11096 - RNA, 19300 nt, Homo sapiens
  source 1..19300: mol_type = other RNA
ctgaatagctgggactacaggtgcacgccaccatgcccggctaattttcgtatcattagtagagacggggtttcaccatattggccaggctggtctcaaactcctgacctcataatcctaattatttactagacttaaatgaagttacatttttatcaaagcataatccaatcaatactgattttaatttaattctatgtcaactaagagggtagactttagcacccgatgtgttgggtttgaatccctggtttttctagatgaatctccttcaaaagcaattgggtcttaaacttttcatatacttgaaatcacaatccatgaagttgctttagtatttcatccctgacaaaccagaaatgagaaatttttaagtttttggaataaaggacaaatacaaagcaggaaatagttttaatttagaaacatctaatcctagataatttagtaacattgattatagcacaattcttgagcactaactatgcaccaggcagtgtttaattgctctgggctcaagcaatcctcttgcctcagcctcccaaattgtggggattataggcgtgagccactgtgcccggccctgggttctttttcttgcattataggaagatgacatttcctggcctcccttgccatgtgacttggacatgtacagtagtgattcatgtctcctccataccaagacagaaaacctcacatcattgcaagtgctttctcttcctcttcatggtggccacgtactaaggtggcagcaacaaaaaaaatggaaggagcccagaaccctgagtcacctgcccgatccacaccaagttgtgatgtgaaggagaaattcagcttgattgtgttactgagtttggggggttgtttgttacagcagctagcatcagttatctcttgtgaaatcacacagctaacaattgagccagtatctgacctagatctattgcctacagagccccacatttaactactattatctggcctctttattgcccccacacacttgaaatataaatttttaaagacattttattcttttttctatccagaatttattgaatcctgatcattttttccttaatgttgattttgtagactcatttccaggaagaacaatgtcaggcagagagaaggaattgaaagagtatttttaataaatttgtacatgttaatataatttacttatttgcaattctcatagctatacgatattctatcccatttccagtgtggcagcgacaaaaaaatggaaggagcctagaaccctgagtcacctacctgacccacaccaggctatgatgtgaaggagaaatacagcttgattgtgttactgagtttggggggttgtttgttacagcagctagcatcaattactctcatacagatgtgtaaacagatacttgcactatagtgttttaggccctgcttcagctcttcctacagtgtcagacatatggtaaccctcatgagttatttgttcagtaaatgatgaatttagaggtagacacatccctttgttacagtgggggtctgaaggagtgttgaggggtgggaaagccacctcactctatgggaaggcgtgtgtactatcgctgatctttccatgtaacaccctttctcctgccaagaatgcccccttttttttttagaagtgcagctaccatatcaaaccatccgctttctggtcccaaagcatgagcagtgcaggcctagctgttaaggtctctcaggtcagataattttatgccttattccccctatcacttcttcagagaaggtaatctttcctagagaaatgtgttctttcgccattgacccctggcagttggtaacattttcaccagcctcctcctattaaactgcagtgatgcagcagcagcccaaagccatagaaaacatggcaaatgtgattttccatgtgtaccaacactcattgctgagcccactttccttgaggccctaaccgtgcacgttcagatagatggcttattattccctgttgtactcggtgtaataaggctagattaatagatttaacttctataaatattcatttattttatcatttccttttagctttgcctctaacaaaacccctaatcttggggtcagggcacctagaaacgtgctcataccctttcatcctgtagatgagtacccttgggtatccatcacaaggaataggatgatagaaaatgagtaacatatgcagagattcagagtatttgctactaaaagagcaaaaacactggaaatgggatagaatatcatatagctatgaaaattgcaaataagtaaatcatattaacatctacaaatttattaaaaatattcattcaattccttctctccacctgacattgttcttcctgcaaatgagtctacaaaatcaacattaaggaaaaaataatcaggattcaataaattctgatgaagacaaaaaagaataaaatgtctttaaaaatttatatttcaagtgtgtggagcaataaggaggcaagataacagtagttaaacgtgcggctctgtaggcaatagatctaggtccagatactggctcaattgttagctgtgtgattttacaagagataatttctttaaacctcagcttttgtttgtttgttttaatctgaaaaatggggataataatgattccggtcttacaggactaaatccgataatatgaaagcagttagcacagtgcttggcacatagaaaatatttaactcagccaggcgtggtggctcatgcctgtaatgccaacagtttgggagaccgaggcgggtggatcacctgaggtcaggagttcaagaccagcctggccaacatggcgaaaccccggctgtactaaaaatacaaaaaaattagctgggtgtggttgtgcgcacttgtagtcccagctgctctggaggctgaggcaggagaatcgcttgaaaccgggaggcagaggttgcggtgagccgaggtcgtggtgagccgaggtcgcgccactgcactccagcctgggagacggagcgggactacgtctcaaaaaaaacaaagcaaacaaacaaacataaaaaatatttaacaagcctgaacttgtttattttttaatatatttatttatttatttattttgagacggagtcccactctatcacccaagctggagtgccgtggcgtgaccttggctcactgcaacctccacctccctggttcaagcaattctcctgcctcagcctcccgaacagctgggactataggcgggcgccaccacacccggctaatttttttgtatttttagtagagatggggtttcgccatgttggccaggctggtctcaaactcctgacctcaggtgatccgcctgtctcggcctcccaaagtgctggcattacaggcgtgagccaccgtgcccggccttaacaagcaacatggtgaaaccccgtctctacaaaaaaatacaaaaactagctgggcatggttgcatgcacctgtaatccctcgtacttgggaggctgaggtgggaggatcacttgagcctgggaggcagaggttgcggtgagccaagatcatgccactgcactccagcctgggtgacagagtgagactctgtctcaaaaaaaagaaaaagaaaaagaaaaaaatatatatatttaacaaatgttaactatttttattatcatatttatgttaacaaatgcacactagaaatggcaatcatttcttccctgggtactgatcacattacatgctcctcctggttttcctcctccgccctggctgctccttctgtctcctctgccagctcctcactccacccaagctctcccaagctgggcttcccagggcttggttatgtgctctgtaccttcctttctctttctctttccgggagtcccatagctttaaatatcaaatttacaccttctggccagaaatcctcccctgagcttcaagtccatctgcctcctagacttctccacttggaagtctaatacctatcttaaattaaataaattcaaacgtgaatacttggttgtacatcctggccaacttcttcctttccccagtcattctttttaagtatatatcaatatattccacccatttgctcaaacaaatactaggagccactcttgattcttttctttctttattcccatatttaatttattagcaaatcttgattttgactctgaaacgaacccccggttcatcccttcctctccttctacctggctatctagtccaagccaccctcatctcctgtgttgctccttaattgtggtctctcacttccctcatgccattccttcccaagctcctccccacccgtggaccccaaacacaactacaacatctacagtgatgtttaaaattgtggttaaaaaattacatagtataaaatttactatcttaaccatgtttaatatgatgttatctgcatgcatattgttggacaacagatctttagaactttttatcttgcaaaactgaaaccctgtaaacactgaacaacaatttccattttcttcctcatcccgatccctggcaatcaccattctgctttctgtttataagagtttgactactttagatatctcatagaagtaaaatcatgcaatgtttgtcctttattgattggctcatttcacttagcttagtatccttaagtttcatccatattgtggcatatgacaggaattccttcttttttaaggctgcataatattctattttatgtgtatggcacattttctttacccattcatccattcatgggttgcttctctcttgtggctattgtgaattaagctgcgtgaacatgagtgtgcaaatatctcttctgttttcaattcttttggatatgtacccagaagtgggcttggtggatcatatgagggttttatttttaattttttgaggaacttccacactgttttccttagtggctctaccattttacattcccaccaacagtgcacaagggtgtcagtttctctacaccctggccaatacttgttattttctggagtttgatcatttgagagtggccatcctaatgggtatgaggtgatatctcattgtggttttgagggtcatcttctaaaaatatagatgctgtcatgttcctttttggaaacttccaatggctttccttgaacttagaatgacatctaagtaccttacttttttttttttttttgagatggagtctcactgtgccgcccaggctgtagtgcagtggcacaatctcgggtcactgcaacctccgtctcatgggttcaagcaattcccctgcttcagcctcccgagtaggtgggattacagttgtgcaccaccaagcccggctaattttaagtaccttactttggcctccaaaatctgatctctgtccacattctggcctttattttcatctccagggcttcttgcttatggtggtacagtcacagtgaatgtgtttgactctttaaccacgtgagcatggtcctgttttcccatgtgcagttccttctgcttgggtctttctcttccttttcacatggctggttccttctcattattcaggtcttagctcaaatgctaccacatccaaggtggcattcaagctgtcccatctaaaatgcttctcctagacactctaaattctatcaccctgtttatttcacttttgctttttgtagcagttatcaacacctgaaattattttgccggtttagctgttggcttatgtagtggtttttttttttttttttttttttttaaatcataccaggaagtacactccatgagaccaggagccctgtgtgtctcattcacagctagatccccggaagggagcctgatttaatgaaaacaaaatgtaacagaacaattaatgccagctgggaggtttggggaacccttcatgaaggatgtaaccattttgttgggtttggaatgatgaatataatttcaacaggcagttgtcaggatgaagtaggggacattttaggctgaggaatgacatgaagtatatgcggagggagcacacagcatcacattttcaaagaaaggtagcttgctatggctgaaactaaaggttccgaagaggaggtggtgagcaggaaggctgaaatggcaggctgaggtcaaagcggcagacattgaattcatttcagttccgccgatttgctatttagttagtgatgcattaggcttgaagatacaaagatgaataagacacagtagtatgccgtcctgcagcagtggggacccacgtgtggcttttgagcagggtaatgacatgagcatgttacagaggtcagaatgcagcagtggttatgagcatagcctccagcaccagatggcgtggaatcaaatcctgctctgtcactatctagctgtgtgaccagggcaagtgtttaactcctgcggcttaattttcttacggataaagatgatgataataactgtggctctcttggctttcttatgagggttaacatttgtagcatggagtctggtactcaatacatgttggctattgacatgcaacgtgttgaggaaaacgatgtcagtacatggtacattttcaatgattgtttgttaggtttctcattttgtttttgagaaagatgatttattggcagcagtgtagataatcatttcaaggaggagacagtgggcacagccacaccaccgtggaagctacggcaatcgttgtggcaaggggaatggtgcacagaattagcttagagcagagataggcagcggaacagattggaggatgtagaggggctgcagaatattttttggaatgaaacaaagtgggtttaatttttgggtctgttgagcttaaggtgcctgaggaaaatctctgtttgctgatgtttagctgaaacaataaagagtcatctgaagtttaggacacagaggtgagtgaaatagagatttgtactctggaaatgtgggtgtgcacattaacaaactgctaagaatttgcattgagcctatcactcacctagtacactggtaaagaaacatgaccatgttttatactcgtgtactgttatgcattactggcagggatgtaaatttgtacaactttgctggaaaacaggtcggcaatatttgtcatgagccttacagataattgcatcctctgacccagtgatttcactttttggagtcaatgctaactttatgatccaaacacagacaattaattattatatacagagctgctcaccacaacataacattcaattgaaaaaaaaacaaaaccttcaaacaggctcactcagtgacaggaaaatggttaaataatgatgtgttcatacgctagaatattatacagccattaaaaaatcatgttgactgagactcctagtgtgaattgctataagggagaaaaacccaatgtatatacaattatatacagaatatgagtttgactctgcttaaaaataacataatgtaaggattagaagacaatatactaagatgttcatattattatttctgtttgggaaatggaggcatgggttggtatttgttgaagtctagtaactgagtttgacttatgactatataatagatttttggcttacttaaaatttcttttccttcttttcctaatgcatctcgtaatatttagttactaacacagtaacaatctttgggcttacagaccaaaattcaaatggcaatttctattacaaatcttgaccatgttttttttttttttttttttttttttgagatagcttctcactcttccacccaggttggagtgcagtggtgcaatcatagcttattgcagcctcaaacatctgggctcaagcaatcttcctgcctcagcctcccaagtacctagtactataggcatgtactactatgtctggctaatttttgtattttttttttttttggtagagatgggatctcacaaaaaaatataaaaattcgcattttttgatcctcctgccttggcctctcaaagtgctgggattacaggcatgagacaccactttttgtttttaatagatgcagtccatcaaaggcccagaacctcaaacttcatttttgagttaatgtcatgtcattgtacaattttgaatgtgccactggaccactgaagatgtttccttctctcctggcttattggcacaatcatccacttgcatttagagggacatgatttttacacaaggggttccttgggtatgtcagagacagaagattagaacaatacaccatcattgagagggtaattcatcaaaagtcctaacttcagctgcacagccaagcagctaaaagaaacccagtgaccctcggaagcacccctgatagacagctgttgggtgtgaaggatccatccataagtcgccagaattggatcgcaaatatcctagagctgacgatctcctggatcatgctgccataactgccttcaagatgttaatactgaacaaggcatgttgtttcagcactgcgggaggagcaatctctcttcccaacccctccgcaccctcccacccacacacgtgcacatgcacacaagcacatgtgttgatatccagcccagtcccatttctcttgctgagactgaccttgatagaaaaactattttgtttttattatagaaggcaagttttctatttactatgtagaaacagataaaaggctactgaagaggtgatgaacctcaccgtgattattaagtgagcaaaaatatttatactaaagtttaaatacttatttgcttatactatagtataagtaagccaaaaattgattatctggtcctaattaattcaaattcgtttactaaacttcaataaattaccaacccatgcctcagtttcccaatattttccagggctatatggcctgtggatagaatttaccatcattctgtgcttttaggacctttttgacattctaggtcaaacttggggaattttcctttttaggagtcccaactactcaaggcagaagccagcaaacacccttgctctgcctttctaagattcttacagggtgcaggcatatgaactgtgggaactgacgaccagttacaccccgttgggactctggttcgggagtgagagatggggaggcaggcgcaattttctcaacaggagatggtcgtggcaggctgaggagcttaagatttgagggtagcaggatggtggagtctttcctggaacaactctacagactgatttgggcatttgttcctggtgggctagcctctaaatccaactctgtggtcctaaagtaggcattgaagaaaaagcatccagcatcgggtaagagaacatgacttgataagcatcaagtaaagcttcaactagtttcagtgtcatctatgaatatttccagtctccatatcagacagtgcttttttggaaagaaagaaaagtatccttgcctttgagtaggccttccggtcaacaggttagttcaacattattccgtcatagtttgggaaaacaattcctttgacaggtgggtccctcaccccccattcatttctccatgtttaaagatatctgcatatactacccaaagtttaatcaggaaatactaaaataaatataatattgagcatattcatgtaatggaattctatatagcagtaaaaatggaaaaaccactattttactaacaatgacgactcttacaaacatacatttcaacaaaaggagccagacacaaaatctacatactgtatgaacccatttatagaaagctaagatgacaggcaaaactacaccatggtgtgattagtcaggatactgatacattcacagaggcatgagcacagtagcttctgggatgctgataatgtgctattgcttaaactgggtggtggatacatcagtgtgtcagctcgtgagaactgttacactaatgatttgcacacttttgttagtattctgcactttaataaaaagtgtttttccttgatttgcctgtcattttttaaactttatatcttatcaatattcaatcttgcacaacttacattgttttacaaagctatctactacatattgctagacctcaagttatcttttttttatatttaaagaaaaatacctggccagatgcaatggctcacacctgtaatcccagcacttgggaggctgaggcaggtagatagatcactttaggtcaggagtttgagaccagcctggccaacatggtgaaaccccgtttccactaaaaatacgaaaagtagctgggtgtggtggcgggtgcctgtaattacagctacttaggaggctgaggcaggagaatcgcttgaatccaggagggggaggttgcagtgagctgagattgcaccactgcactacagcctgggtgacacagagagattcgtctcaaaaaaaaaaaaaaaaaagtaaagaaaaataccaatacacggggagttctaagcacagaaaaataacctaaggattatttttcaatttattcaaatgaaaccaaagatgggcttgccgtggttaactagagtctttctcaaaagaaagatttcaatctggtgtatgtttaggaggcttgtacactctcagcttctcagttaagtgtctgccaagactcttttctctgactacacattgagcctccaaaccatgactgaaaaaccacagcttcatgggcagggccctgtgcaggacaccctatttccaaatgaacaagaaatgaaagtgagataaaaaaatattttaaaggtaaaagtttcacattatttaatgcaagctagctgtcaaggagaaagtagtgatgaatgaaaggaaaggaacaaagacaccacagagatgcacatcaaactggaagcagacaaaggcagccagaactatcttatttattataaagatacaccgtgaagaacaaacctgactgtatactgaagcctgtaatggtacatgccaaaaatgtacagtactatacataaaagtgcattgtcacaacagattaacaaaacattttttttctttccagactgtaaaagcatccccctttattttcacctcagagaggagggaatgaaatggtgagaggcagtacagagcacgggcgaatgcgatgctgtcagcagcacatgagcgggggactgatgcggtgggatgggaggacacaggggtgagaaaggcacaatcacgtctacaaggaaaacgagacagtctgaggaccgacagggaggtgagatgggacattactgagcaccgaggcacaggaaggcggggatggggaaggtgggggacagggaggaagcttcgaaacactcgagtgggcagcaggaattgggaggaggaggtgggggtggggcacagagcggggcaacggtacaagagcaaggctaaaactcctctaaaatagaaaggcactttcacatgtacatactacagatgtacattgacacaattaggtaacagtcacaagcaggaagctaccggtaccgcaattgatcaaaccgacaggaaaggacaatactgatttaattacgcgggcagcagttacccttcagtacgtaggtaaacagcagtctctcctgttacacagccacttactatactttaaatatctataataaccatcacactacacactgaacttggatgaatgctctaaggggggcattcacaaatgcacggttcatatattttcttttactaaagtttctaagataagcattatggaacccagtacaattatttaaacatacaaaattccctacgtaatttaaagacacaggtatccatctcgattataccacatagacttttttttttttttaagaacgtatactagggtaagtgaaagctcaaattccagtttgctttatggatctgacaaaacttcgccaaagtcaccctgcaccaagcctgactctccagcccagctggagcttgtgttctcaacttgggaggtgggtggcaggtggtctggagtagggagctctatttacgcctgggtagagacttctaagctgctctgtgtctcagggtttctgtggtggataatcgaaaacaagactgagtcctaagcacatttcctgcacaaaaaatggcctctcactgctatggtcaggaatcaatgagcatcatcccaaatttgaatcctctaacccccgcctcaagagacacataggctctttaactttggatttccaaggctgatcagatgaaagtttcttcagtttgtagactccagaggctatgtcattcctaaatgttaaggacacaactaccaacccacgcctcttttccttttctttaaattataaaccccccctttttttggtcgcgggggggatagcaaaagttagaaaacccttaacggatacaatttgactcttggagcactatatccactgataactgttcacgatcattgcagtagattgtgggaccctgctataaattattctacaggtggctcaaggggcaccaaagccagattatgttgtacgaagatgtgcaaagctgttgaatggtgttgacactgaacgtgaacatggagctctacaaagcgccactcagcaggttcaaacagttcacgtaacgcccattagaaaatgtgtactaagtacacctttctctctatccccaaatccactccccaaaccccaacccagtccaaaaggctgacttgatgaatctccttcagtgagttctatggatgggatgtgaacacacagttatatcagctgagaatacatattcttgtgtcagtggagtcaggtaatctttgtagagccattatttacccaccatcaaaaagctcccctccccaaattgcacatgaagcctgataagctccttgaaattgggggcagaacacctcaaggcctcattatccttcttctctcgtttccctgtgtcttcccacctcccctgtgtgctgcctctgtggctataaagaagggctgtgaaccttctcagctgcagtggcttttaatgagctttactgagcatgattctggattctttgtgaagtggccaccttgtcttatctctggaatctgaagacatttaataaaccaagtaaggagaggtgagtctttactgagtcctcactcactctgaggtcatacccttcatttggaattgaaaaaaaaaaaaagtctcaagctgacaataggagtatagggaaataagatggagacaggtaaagtgagtgatgggagagtattaggagctgtttcctgaaacaaggcacagcctgtgaggctctgcagcagcacgactcctgccggccaagacagcaaagtcctgatggggagcacagaaaggcaatcctcgttccaccgtaggtggacacatcagagagaggagccgctggggaggatgaccagatagaaggctgaataaatgaacaggtaggaggaagatctgaaaagctaaggctgaagctcagaaaagacattgaaaaaaaataaattcaaagacacctctggccctttgatgccctctgttaacatcttactcttccatcaaacaaggaatatggtttttaagaattcttactattttaaagaagtggtggaatggccgggcatggtggctcacatctgtaatcccagcactttgggaggctgaggctggtgggtcacctgaggtcaggagtttgagaccagcctggccaacatggtgacaccccatctctactaaaaatacaaaaattagctgggcgtggtggtggcgcctgtaatcccagctactcaggagaattgcttgaacccgggagatggaggttgcagggagccgagattgcaccactgtactctggcctgggcgacagagcaagactccaactcaaaaaaaaaaaaaaaaaaaaaaaaaagtgggggattattttggaaagtttaaattcctaaggaatttgtgaggattgtttaaaagggctagtgctattcaaagctcagtcttggctggatctccacggtgtccaagggtgctgaaggaccccaaaagctcaggagaaatggggaggggctagacaaggtgctgtcctgggcttctttttcaaaatgggcaaaaagtatggctctgaaaatttggaggtttaaaagtttaccatacctagaaatacatgggaaaaaagtcactattcatttgtgaaattaggccccaggcaagcaatcagcagtgtgactctgaaagtaacaatatctcatcaatttaatctcttcctgcaatagaatgactacactggcaaactgaggtagagatcaaagtaatgatcttgattttagtacagatcccagttcttttctgcacgatgcattcaccaatgggctgatgaagtaaaatctacactgtgtagctcttagatgggcgtgcaattggctgccagtttgaaatgaaaccaagaaggaaattaatggtgggccagagggattagttgtgggaaatccatttctcccaacaacaacaacaacaacaaaaatctttatcagtaacttcaatgatagaatagataaaatgctcataggtctacaggtgatatcagctgctgctagtaggagaatggaaatcaaagcaaattttcttaagatgggggaaaatgtagcataaatataggcttaaaaaattgcctgtgtgctaggatgccagagaaagagggtctccaattgagagttcagctgactatgggagttacatagagcccacatacaaaaccaaaaccaaaaaggggaaaagggacaaagaaaaagaagttgtggttgtgaggtacacaactgggtgagaaccacaaggccatgttctgctgatggccctgcatggctcttactcaggtaccagggccagttcagggttggctcaaagacaaatggagaggacagttgggatttcaaatttaggatcatcaggactttgtagcattttttttttttttaagagacagggtctcacactatgctgcccaggctggactcgaactactaggcccaaagccatcctcctgtgtaaaccacccgagtagctgggagtacaggtgtgcaccaccatgcctgggctttgtagcatgtttaaaggaacctaggtgatttagtcaaaagagaacactgcatgaaccaaggcctcaggtgcttcttgctgccttcatttccacagaggagaacacagggatttagaggagatggaaacattttctaggcagttattgaataacggatctttggaggagttcgtggagtagtgtaaccagaaagtctttaaaattaaacccttctaatcgtttgtaagtgtagatggggggacttggaaatctccggggcctaatcatgctcgcaaaaggagtgacattaatagctttggagatggtgtcttcctctcctttcccaggttaagttcaagcagtaacagcagaggttctacctccttccatcgagtctttaagctggacccggggaaataactgttaggaaagaggcaagcatccaacccactcgagctgtgggctgacagtcccactgggatcgtcccatggagacaattgcaagtcttttgcatgagctaaaccccgctccacatggaaccgaaggtgctcattgtcagctaccacgcaatgccattatcacctttcagcccaagtgccacagaccaacactggctatactccaatgaggtgtggcattcgggttcttctgccttcaggtcacaacctttctgactcagctgggctacattaaacctgaagctctgtacaatgtggagagcggtgttgccttcattacaagtggtgcagcattggattttcaagtaagtctaagtgtttctattgtccttaaaatgacatatgtccagttatttaaaaaaattacaaaatacaaatgcccgtgttaatttagctagtctcagacattacattcgacaacatagaaaagccaaaagatctccagttataagcacaaaactaaggaaagttatggatcagtgacttttgtcactaatccattttcttttttaagtcacctccctttatggccttgcttggctggtttttacattgtgcatgacttgtctgttggaccctggggaggtggggcaggtcctatggtaggatttgtttttggaagaacagcaggttttggcctaagggctggaggcttcagctgcacgcccattctgggtgccaccataggcttgaaagtactcattgtgtcactggaggagctcgtgctacgtcgaatctgaggctcggagctcctgagggcaacgttgtgcaaagggctgagagattccgtggaagtggcaggggtgggagagtttttcacttgctccagggtatccagcaccacatcaggggcatgctttgctgtgctctgtctctccagttctcggagttcattcaaagctgtgttcatcgtttcttcaatatcctgagcaattgtctctgggtccagtggcttgtggtcattgaagcccgtgtattgccctgatgacgtggaccttctaatgggagggctgtcgatcttcttgagggagtcgtgccggctgatgttggtcaggctgccatggccaggcctgcgcctccgctcaggactgtcattgttgaggccacggttctgcagcaggccccgggggtgactggcaaggcttggggaccctaggtcaactgaggagttagaaagggcatgtggagggtggagcgggcaatggccatcactggtcctgccaggacgccttactggagggggtggctctcctctttttcgttgcctggctaaatagccgtcaggatgacggtctgtcggggagttcatgtccttggatgaggacttgtcttccgtgactggcccactgctggcctcactgtcggctttttggctcagagtgtctgaaaacgtatcatccatatcctgcaccactatatactggtgaggcaccagcccgtcaatcccgttgtgcctgccttcccaccagtcctcagatgcacggtgatacagcagcagggaggcacccttcttgaaggatagttctctggcagaccgcccaacatagtcaaacttggctattgcttctattggctcacattcatcttcacttgtgtggggctctgtaccagcatcttggtccacttcctccaatgtaccgtgctcactgtatgggctgtcgcaatagtcatctccagccatacatttctcataaacagggccatccagctctttagcatctgggaaaatagtctcatggtggatgatgatggttttgataatttcattcacatgtgcctggcaagacacttgatcctgtatttctgggacaggcatcaatgttgggccaaagcaaatggccaggttataagggtccatcatattctcatcgctgtactgtgatagatgattgaggaaggcaaagaggtacctcatcactataaggaccgacctgggcaaagtcaggaggagtttgcggatgtgaagcgccctctcatagagattatctattctgatacaagaaatcagatcgttaaatctttccttaggaaagagggggttttccagcccacggaaatagagcttcagaacgccagcaactgagttaatatcatggttactctggtcatcagccaaaggattttcacctctctcaaatgaatttttaatatcattgacttccacctgggaaccagacactctgaaaatcccctgatgctgaagaccatagagattgatgaaccgaatacagctttccacaatgaggggaataacctgtcctgagtcctgatgtcttgtgtgcgagtttcttcgtcctcggcttgtagtcatatattcagctctatgaccttctcccagggtcctctgcagcaagtcatgtttggcttgaagttttgtgatgagattactgccttccaaatattctctgagtttcatgaagtagaactgttcagtttcctgctggttggctcttctcttggcgatgctgggtttactcaggtaggtttcagagacagtggacttcactgattctgtggaacgactgtgctggaagcattcagaaacatcatagtcctcgatggtgaccatatcttgtatcgtctgcaaggtggcttcagtcgttttcttaacctcttcattctcgattttgagcgtggcaaggcgggactgcaactgttggtacctgagcatgagctctgcctggactggctgctgggcactgacctggcacacctcatcacccatgtgagactgaaactcaaacttcattggtggacagaacgcagcagggtacatctccatgaatctctgcttatcgctcctgggctctaaattatcaactgcattctcaataatgtctaagccctcatgtctggaggtttcaaggttgtactccgcagacagatatgttcttagggctctgttcagacttgcatggtagccaagatcacagcaatcaattaaatcagaaagatcatgaatatagtacttgaaaactgaggcattggtggcttcaagtgttaggagatattcgttccgtgccttaattgattttagcttattttctgaatattttgcttgtcttttttctttcattttttcaattttctttacagagcttcgccgttgatgtctctcctctagtcgaatatggaagactggatcaccagatctcccaatttgcttttcctcttgtttttcggcctctttcagcttgctctctgcactgatgctctctgcatgatacatatggtatgttttcatcaccgtataaagctcattaagaaccttcattaaatcctcatgaagttggaatgcaatctctttgctctttttaaacatcctggtagaatcctcacttatctgcatgaaccgcataatcacattgttcagatagatgtcactcaaggttgcatggtctttgctttctctccttacttggttcaggagcaaataccagcagttcactggagacaacaggttctggtctttcttgtattgttgatgatccttagtgcttcttgtttttgccatgaacctttctgctaacttctctagattccgggaatattccgtctcaatttcagctttttttcggaagaaatcttgcagatcctggagaagctgaactcgcatctccgtttgctgctccaggcatttttgttgttctaccagttgagctcgaatttctttgacttgactttcatactcggctatgatctctttgtccttcttgaatcggctcggggtggacattatccagctgttccgggtttgctttcaatgggcaagttttgttcagtggtcacaacccgttctccttggagaggcagagttgtactcccacacgcaggcaatccagaggcagcgccg

SEQ ID NO: 11097 - RNA, 19369 nt, Homo sapiens
  source 1..19369: mol_type = other RNA
ctgaatagctgggactacaggtgcacgccaccatgcccggctaattttcgtatcattagtagagacggggtttcaccatattggccaggctggtctcaaactcctgacctcataatcctaattatttactagacttaaatgaagttacatttttatcaaagcataatccaatcaatactgattttaatttaattctatgtcaactaagagggtagactttagcacccgatgtgttgggtttgaatccctggtttttctagatgaatctccttcaaaagcaattgggtcttaaacttttcatatacttgaaatcacaatccatgaagttgctttagtatttcatccctgacaaaccagaaatgagaaatttttaagtttttggaataaaggacaaatacaaagcaggaaatagttttaatttagaaacatctaatcctagataatttagtaacattgattatagcacaattcttgagcactaactatgcaccaggcagtgtttaattgctctgggctcaagcaatcctcttgcctcagcctcccaaattgtggggattataggcgtgagccactgtgcccggccctgggttctttttcttgcattataggaagatgacatttcctggcctcccttgccatgtgacttggacatgtacagtagtgattcatgtctcctccataccaagacagaaaacctcacatcattgcaagtgctttctcttcctcttcatggtggccacgtactaaggtggcagcaacaaaaaaaatggaaggagcccagaaccctgagtcacctgcccgatccacaccaagttgtgatgtgaaggagaaattcagcttgattgtgttactgagtttggggggttgtttgttacagcagctagcatcagttatctcttgtgaaatcacacagctaacaattgagccagtatctgacctagatctattgcctacagagccccacatttaactactattatctggcctctttattgcccccacacacttgaaatataaatttttaaagacattttattcttttttctatccagaatttattgaatcctgatcattttttccttaatgttgattttgtagactcatttccaggaagaacaatgtcaggcagagagaaggaattgaaagagtatttttaataaatttgtacatgttaatataatttacttatttgcaattctcatagctatacgatattctatcccatttccagtgtggcagcgacaaaaaaatggaaggagcctagaaccctgagtcacctacctgacccacaccaggctatgatgtgaaggagaaatacagcttgattgtgttactgagtttggggggttgtttgttacagcagctagcatcaattactctcatacagatgtgtaaacagatacttgcactatagtgttttaggccctgcttcagctcttcctacagtgtcagacatatggtaaccctcatgagttatttgttcagtaaatgatgaatttagaggtagacacatccctttgttacagtgggggtctgaaggagtgttgaggggtgggaaagccacctcactctatgggaaggcgtgtgtactatcgctgatctttccatgtaacaccctttctcctgccaagaatgcccccttttttttttagaagtgcagctaccatatcaaaccatccgctttctggtcccaaagcatgagcagtgcaggcctagctgttaaggtctctcaggtcagataattttatgccttattccccctatcacttcttcagagaaggtaatctttcctagagaaatgtgttctttcgccattgacccctggcagttggtaacattttcaccagcctcctcctattaaactgcagtgatgcagcagcagcccaaagccatagaaaacatggcaaatgtgattttccatgtgtaccaacactcattgctgagcccactttccttgaggccctaaccgtgcacgttcagatagatggcttattattccctgttgtactcggtgtaataaggctagattaatagatttaacttctataaatattcatttattttatcatttccttttagctttgcctctaacaaaacccctaatcttggggtcagggcacctagaaacgtgctcataccctttcatcctgtagatgagtacccttgggtatccatcacaaggaataggatgatagaaaatgagtaacatatgcagagattcagagtatttgctactaaaagagcaaaaacactggaaatgggatagaatatcatatagctatgaaaattgcaaataagtaaatcatattaacatctacaaatttattaaaaatattcattcaattccttctctccacctgacattgttcttcctgcaaatgagtctacaaaatcaacattaaggaaaaaataatcaggattcaataaattctgatgaagacaaaaaagaataaaatgtctttaaaaatttatatttcaagtgtgtggagcaataaggaggcaagataacagtagttaaacgtgcggctctgtaggcaatagatctaggtccagatactggctcaattgttagctgtgtgattttacaagagataatttctttaaacctcagcttttgtttgtttgttttaatctgaaaaatggggataataatgattccggtcttacaggactaaatccgataatatgaaagcagttagcacagtgcttggcacatagaaaatatttaactcagccaggcgtggtggctcatgcctgtaatgccaacagtttgggagaccgaggcgggtggatcacctgaggtcaggagttcaagaccagcctggccaacatggcgaaaccccggctgtactaaaaatacaaaaaaattagctgggtgtggttgtgcgcacttgtagtcccagctgctctggaggctgaggcaggagaatcgcttgaaaccgggaggcagaggttgcggtgagccgaggtcgtggtgagccgaggtcgcgccactgcactccagcctgggagacggagcgggactacgtctcaaaaaaaacaaagcaaacaaacaaacataaaaaatatttaacaagcctgaacttgtttattttttaatatatttatttatttatttattttgagacggagtcccactctatcacccaagctggagtgccgtggcgtgaccttggctcactgcaacctccacctccctggttcaagcaattctcctgcctcagcctcccgaacagctgggactataggcgggcgccaccacacccggctaatttttttgtatttttagtagagatggggtttcgccatgttggccaggctggtctcaaactcctgacctcaggtgatccgcctgtctcggcctcccaaagtgctggcattacaggcgtgagccaccgtgcccggccttaacaagcaacatggtgaaaccccgtctctacaaaaaaatacaaaaactagctgggcatggttgcatgcacctgtaatccctcgtacttgggaggctgaggtgggaggatcacttgagcctgggaggcagaggttgcggtgagccaagatcatgccactgcactccagcctgggtgacagagtgagactctgtctcaaaaaaaagaaaaagaaaaagaaaaaaatatatatatttaacaaatgttaactatttttattatcatatttatgttaacaaatgcacactagaaatggcaatcatttcttccctgggtactgatcacattacatgctcctcctggttttcctcctccgccctggctgctccttctgtctcctctgccagctcctcactccacccaagctctcccaagctgggcttcccagggcttggttatgtgctctgtaccttcctttctctttctctttccgggagtcccatagctttaaatatcaaatttacaccttctggccagaaatcctcccctgagcttcaagtccatctgcctcctagacttctccacttggaagtctaatacctatcttaaattaaataaattcaaacgtgaatacttggttgtacatcctggccaacttcttcctttccccagtcattctttttaagtatatatcaatatattccacccatttgctcaaacaaatactaggagccactcttgattcttttctttctttattcccatatttaatttattagcaaatcttgattttgactctgaaacgaacccccggttcatcccttcctctccttctacctggctatctagtccaagccaccctcatctcctgtgttgctccttaattgtggtctctcacttccctcatgccattccttcccaagctcctccccacccgtggaccccaaacacaactacaacatctacagtgatgtttaaaattgtggttaaaaaattacatagtataaaatttactatcttaaccatgtttaatatgatgttatctgcatgcatattgttggacaacagatctttagaactttttatcttgcaaaactgaaaccctgtaaacactgaacaacaatttccattttcttcctcatcccgatccctggcaatcaccattctgctttctgtttataagagtttgactactttagatatctcatagaagtaaaatcatgcaatgtttgtcctttattgattggctcatttcacttagcttagtatccttaagtttcatccatattgtggcatatgacaggaattccttcttttttaaggctgcataatattctattttatgtgtatggcacattttctttacccattcatccattcatgggttgcttctctcttgtggctattgtgaattaagctgcgtgaacatgagtgtgcaaatatctcttctgttttcaattcttttggatatgtacccagaagtgggcttggtggatcatatgagggttttatttttaattttttgaggaacttccacactgttttccttagtggctctaccattttacattcccaccaacagtgcacaagggtgtcagtttctctacaccctggccaatacttgttattttctggagtttgatcatttgagagtggccatcctaatgggtatgaggtgatatctcattgtggttttgagggtcatcttctaaaaatatagatgctgtcatgttcctttttggaaacttccaatggctttccttgaacttagaatgacatctaagtaccttacttttttttttttttttgagatggagtctcactgtgccgcccaggctgtagtgcagtggcacaatctcgggtcactgcaacctccgtctcatgggttcaagcaattcccctgcttcagcctcccgagtaggtgggattacagttgtgcaccaccaagcccggctaattttaagtaccttactttggcctccaaaatctgatctctgtccacattctggcctttattttcatctccagggcttcttgcttatggtggtacagtcacagtgaatgtgtttgactctttaaccacgtgagcatggtcctgttttcccatgtgcagttccttctgcttgggtctttctcttccttttcacatggctggttccttctcattattcaggtcttagctcaaatgctaccacatccaaggtggcattcaagctgtcccatctaaaatgcttctcctagacactctaaattctatcaccctgtttatttcacttttgctttttgtagcagttatcaacacctgaaattattttgccggtttagctgttggcttatgtagtggtttttttttttttttttttttttttaaatcataccaggaagtacactccatgagaccaggagccctgtgtgtctcattcacagctagatccccggaagggagcctgatttaatgaaaacaaaatgtaacagaacaattaatgccagctgggaggtttggggaacccttcatgaaggatgtaaccattttgttgggtttggaatgatgaatataatttcaacaggcagttgtcaggatgaagtaggggacattttaggctgaggaatgacatgaagtatatgcggagggagcacacagcatcacattttcaaagaaaggtagcttgctatggctgaaactaaaggttccgaagaggaggtggtgagcaggaaggctgaaatggcaggctgaggtcaaagcggcagacattgaattcatttcagttccgccgatttgctatttagttagtgatgcattaggcttgaagatacaaagatgaataagacacagtagtatgccgtcctgcagcagtggggacccacgtgtggcttttgagcagggtaatgacatgagcatgttacagaggtcagaatgcagcagtggttatgagcatagcctccagcaccagatggcgtggaatcaaatcctgctctgtcactatctagctgtgtgaccagggcaagtgtttaactcctgcggcttaattttcttacggataaagatgatgataataactgtggctctcttggctttcttatgagggttaacatttgtagcatggagtctggtactcaatacatgttggctattgacatgcaacgtgttgaggaaaacgatgtcagtacatggtacattttcaatgattgtttgttaggtttctcattttgtttttgagaaagatgatttattggcagcagtgtagataatcatttcaaggaggagacagtgggcacagccacaccaccgtggaagctacggcaatcgttgtggcaaggggaatggtgcacagaattagcttagagcagagataggcagcggaacagattggaggatgtagaggggctgcagaatattttttggaatgaaacaaagtgggtttaatttttgggtctgttgagcttaaggtgcctgaggaaaatctctgtttgctgatgtttagctgaaacaataaagagtcatctgaagtttaggacacagaggtgagtgaaatagagatttgtactctggaaatgtgggtgtgcacattaacaaactgctaagaatttgcattgagcctatcactcacctagtacactggtaaagaaacatgaccatgttttatactcgtgtactgttatgcattactggcagggatgtaaatttgtacaactttgctggaaaacaggtcggcaatatttgtcatgagccttacagataattgcatcctctgacccagtgatttcactttttggagtcaatgctaactttatgatccaaacacagacaattaattattatatacagagctgctcaccacaacataacattcaattgaaaaaaaaacaaaaccttcaaacaggctcactcagtgacaggaaaatggttaaataatgatgtgttcatacgctagaatattatacagccattaaaaaatcatgttgactgagactcctagtgtgaattgctataagggagaaaaacccaatgtatatacaattatatacagaatatgagtttgactctgcttaaaaataacataatgtaaggattagaagacaatatactaagatgttcatattattatttctgtttgggaaatggaggcatgggttggtatttgttgaagtctagtaactgagtttgacttatgactatataatagatttttggcttacttaaaatttcttttccttcttttcctaatgcatctcgtaatatttagttactaacacagtaacaatctttgggcttacagaccaaaattcaaatggcaatttctattacaaatcttgaccatgttttttttttttttttttttttttttgagatagcttctcactcttccacccaggttggagtgcagtggtgcaatcatagcttattgcagcctcaaacatctgggctcaagcaatcttcctgcctcagcctcccaagtacctagtactataggcatgtactactatgtctggctaatttttgtattttttttttttttggtagagatgggatctcacaaaaaaatataaaaattcgcattttttgatcctcctgccttggcctctcaaagtgctgggattacaggcatgagacaccactttttgtttttaatagatgcagtccatcaaaggcccagaacctcaaacttcatttttgagttaatgtcatgtcattgtacaattttgaatgtgccactggaccactgaagatgtttccttctctcctggcttattggcacaatcatccacttgcatttagagggacatgatttttacacaaggggttccttgggtatgtcagagacagaagattagaacaatacaccatcattgagagggtaattcatcaaaagtcctaacttcagctgcacagccaagcagctaaaagaaacccagtgaccctcggaagcacccctgatagacagctgttgggtgtgaaggatccatccataagtcgccagaattggatcgcaaatatcctagagctgacgatctcctggatcatgctgccataactgccttcaagatgttaatactgaacaaggcatgttgtttcagcactgcgggaggagcaatctctcttcccaacccctccgcaccctcccacccacacacgtgcacatgcacacaagcacatgtgttgatatccagcccagtcccatttctcttgctgagactgaccttgatagaaaaactattttgtttttattatagaaggcaagttttctatttactatgtagaaacagataaaaggctactgaagaggtgatgaacctcaccgtgattattaagtgagcaaaaatatttatactaaagtttaaatacttatttgcttatactatagtataagtaagccaaaaattgattatctggtcctaattaattcaaattcgtttactaaacttcaataaattaccaacccatgcctcagtttcccaatattttccagggctatatggcctgtggatagaatttaccatcattctgtgcttttaggacctttttgacattctaggtcaaacttggggaattttcctttttaggagtcccaactactcaaggcagaagccagcaaacacccttgctctgcctttctaagattcttacagggtgcaggcatatgaactgtgggaactgacgaccagttacaccccgttgggactctggttcgggagtgagagatggggaggcaggcgcaattttctcaacaggagatggtcgtggcaggctgaggagcttaagatttgagggtagcaggatggtggagtctttcctggaacaactctacagactgatttgggcatttgttcctggtgggctagcctctaaatccaactctgtggtcctaaagtaggcattgaagaaaaagcatccagcatcgggtaagagaacatgacttgataagcatcaagtaaagcttcaactagtttcagtgtcatctatgaatatttccagtctccatatcagacagtgcttttttggaaagaaagaaaagtatccttgcctttgagtaggccttccggtcaacaggttagttcaacattattccgtcatagtttgggaaaacaattcctttgacaggtgggtccctcaccccccattcatttctccatgtttaaagatatctgcatatactacccaaagtttaatcaggaaatactaaaataaatataatattgagcatattcatgtaatggaattctatatagcagtaaaaatggaaaaaccactattttactaacaatgacgactcttacaaacatacatttcaacaaaaggagccagacacaaaatctacatactgtatgaacccatttatagaaagctaagatgacaggcaaaactacaccatggtgtgattagtcaggatactgatacattcacagaggcatgagcacagtagcttctgggatgctgataatgtgctattgcttaaactgggtggtggatacatcagtgtgtcagctcgtgagaactgttacactaatgatttgcacacttttgttagtattctgcactttaataaaaagtgtttttccttgatttgcctgtcattttttaaactttatatcttatcaatattcaatcttgcacaacttacattgttttacaaagctatctactacatattgctagacctcaagttatcttttttttatatttaaagaaaaatacctggccagatgcaatggctcacacctgtaatcccagcacttgggaggctgaggcaggtagatagatcactttaggtcaggagtttgagaccagcctggccaacatggtgaaaccccgtttccactaaaaatacgaaaagtagctgggtgtggtggcgggtgcctgtaattacagctacttaggaggctgaggcaggagaatcgcttgaatccaggagggggaggttgcagtgagctgagattgcaccactgcactacagcctgggtgacacagagagattcgtctcaaaaaaaaaaaaaaaaaagtaaagaaaaataccaatacacggggagttctaagcacagaaaaataacctaaggattatttttcaatttattcaaatgaaaccaaagatgggcttgccgtggttaactagagtctttctcaaaagaaagatttcaatctggtgtatgtttaggaggcttgtacactctcagcttctcagttaagtgtctgccaagactcttttctctgactacacattgagcctccaaaccatgactgaaaaaccacagcttcatgggcagggccctgtgcaggacaccctatttccaaatgaacaagaaatgaaagtgagataaaaaaatattttaaaggtaaaagtttcacattatttaatgcaagctagctgtcaaggagaaagtagtgatgaatgaaaggaaaggaacaaagacaccacagagatgcacatcaaactggaagcagacaaaggcagccagaactatcttatttattataaagatacaccgtgaagaacaaacctgactgtatactgaagcctgtaatggtacatgccaaaaatgtacagtactatacataaaagtgcattgtcacaacagattaacaaaacattttttttctttccagactgtaaaagcatccccctttattttcacctcagagaggagggaatgaaatggtgagaggcagtacagagcacgggcgaatgcgatgctgtcagcagcacatgagcgggggactgatgcggtgggatgggaggacacaggggtgagaaaggcacaatcacgtctacaaggaaaacgagacagtctgaggaccgacagggaggtgagatgggacattactgagcaccgaggcacaggaaggcggggatggggaaggtgggggacagggaggaagcttcgaaacactcgagtgggcagcaggaattgggaggaggaggtgggggtggggcacagagcggggcaacggtacaagagcaaggctaaaactcctctaaaatagaaaggcactttcacatgtacatactacagatgtacattgacacaattaggtaacagtcacaagcaggaagctaccggtaccgcaattgatcaaaccgacaggaaaggacaatactgatttaattacgcgggcagcagttacccttcagtacgtaggtaaacagcagtctctcctgttacacagccacttactatactttaaatatctataataaccatcacactacacactgaacttggatgaatgctctaaggggggcattcacaaatgcacggttcatatattttcttttactaaagtttctaagataagcattatggaacccagtacaattatttaaacatacaaaattccctacgtaatttaaagacacaggtatccatctcgattataccacatagacttttttttttttttaagaacgtatactagggtaagtgaaagctcaaattccagtttgctttatggatctgacaaaacttcgccaaagtcaccctgcaccaagcctgactctccagcccagctggagcttgtgttctcaacttgggaggtgggtggcaggtggtctggagtagggagctctatttacgcctgggtagagacttctaagctgctctgtgtctcagggtttctgtggtggataatcgaaaacaagactgagtcctaagcacatttcctgcacaaaaaatggcctctcactgctatggtcaggaatcaatgagcatcatcccaaatttgaatcctctaacccccgcctcaagagacacataggctctttaactttggatttccaaggctgatcagatgaaagtttcttcagtttgtagactccagaggctatgtcattcctaaatgttaaggacacaactaccaacccacgcctcttttccttttctttaaattataaaccccccctttttttggtcgcgggggggatagcaaaagttagaaaacccttaacggatacaatttgactcttggagcactatatccactgataactgttcacgatcattgcagtagattgtgggaccctgctataaattattctacaggtggctcaaggggcaccaaagccagattatgttgtacgaagatgtgcaaagctgttgaatggtgttgacactgaacgtgaacatggagctctacaaagcgccactcagcaggttcaaacagttcacgtaacgcccattagaaaatgtgtactaagtacacctttctctctatccccaaatccactccccaaaccccaacccagtccaaaaggctgacttgatgaatctccttcagtgagttctatggatgggatgtgaacacacagttatatcagctgagaatacatattcttgtgtcagtggagtcaggtaatctttgtagagccattatttacccaccatcaaaaagctcccctccccaaattgcacatgaagcctgataagctccttgaaattgggggcagaacacctcaaggcctcattatccttcttctctcgtttccctgtgtcttcccacctcccctgtgtgctgcctctgtggctataaagaagggctgtgaaccttctcagctgcagtggcttttaatgagctttactgagcatgattctggattctttgtgaagtggccaccttgtcttatctctggaatctgaagacatttaataaaccaagtaaggagaggtgagtctttactgagtcctcactcactctgaggtcatacccttcatttggaattgaaaaaaaaaaaaagtctcaagctgacaataggagtatagggaaataagatggagacaggtaaagtgagtgatgggagagtattaggagctgtttcctgaaacaaggcacagcctgtgaggctctgcagcagcacgactcctgccggccaagacagcaaagtcctgatggggagcacagaaaggcaatcctcgttccaccgtaggtggacacatcagagagaggagccgctggggaggatgaccagatagaaggctgaataaatgaacaggtaggaggaagatctgaaaagctaaggctgaagctcagaaaagacattgaaaaaaaataaattcaaagacacctctggccctttgatgccctctgttaacatcttactcttccatcaaacaaggaatatggtttttaagaattcttactattttaaagaagtggtggaatggccgggcatggtggctcacatctgtaatcccagcactttgggaggctgaggctggtgggtcacctgaggtcaggagtttgagaccagcctggccaacatggtgacaccccatctctactaaaaatacaaaaattagctgggcgtggtggtggcgcctgtaatcccagctactcaggagaattgcttgaacccgggagatggaggttgcagggagccgagattgcaccactgtactctggcctgggcgacagagcaagactccaactcaaaaaaaaaaaaaaaaaaaaaaaaaagtgggggattattttggaaagtttaaattcctaaggaatttgtgaggattgtttaaaagggctagtgctattcaaagctcagtcttggctggatctccacggtgtccaagggtgctgaaggaccccaaaagctcaggagaaatggggaggggctagacaaggtgctgtcctgggcttctttttcaaaatgggcaaaaagtatggctctgaaaatttggaggtttaaaagtttaccatacctagaaatacatgggaaaaaagtcactattcatttgtgaaattaggccccaggcaagcaatcagcagtgtgactctgaaagtaacaatatctcatcaatttaatctcttcctgcaatagaatgactacactggcaaactgaggtagagatcaaagtaatgatcttgattttagtacagatcccagttcttttctgcacgatgcattcaccaatgggctgatgaagtaaaatctacactgtgtagctcttagatgggcgtgcaattggctgccagtttgaaatgaaaccaagaaggaaattaatggtgggccagagggattagttgtgggaaatccatttctcccaacaacaacaacaacaacaaaaatctttatcagtaacttcaatgatagaatagataaaatgctcataggtctacaggtgatatcagctgctgctagtaggagaatggaaatcaaagcaaattttcttaagatgggggaaaatgtagcataaatataggcttaaaaaattgcctgtgtgctaggatgccagagaaagagggtctccaattgagagttcagctgactatgggagttacatagagcccacatacaaaaccaaaaccaaaaaggggaaaagggacaaagaaaaagaagttgtggttgtgaggtacacaactgggtgagaaccacaaggccatgttctgctgatggccctgcatggctcttactcaggtaccagggccagttcagggttggctcaaagacaaatggagaggacagttgggatttcaaatttaggatcatcaggactttgtagcattttttttttttttaagagacagggtctcacactatgctgcccaggctggactcgaactactaggcccaaagccatcctcctgtgtaaaccacccgagtagctgggagtacaggtgtgcaccaccatgcctgggctttgtagcatgtttaaaggaacctaggtgatttagtcaaaagagaacactgcatgaaccaaggcctcaggtgcttcttgctgccttcatttccacagaggagaacacagggatttagaggagatggaaacattttctaggcagttattgaataacggatctttggaggagttcgtggagtagtgtaaccagaaagtctttaaaattaaacccttctaatcgtttgtaagtgtagatggggggacttggaaatctccggggcctaatcatgctcgcaaaaggagtgacattaatagctttggagatggtgtcttcctctcctttcccaggttaagttcaagcagtaacagcagaggttctacctccttccatcgagtctttaagctggacccggggaaataactgttaggaaagaggcaagcatccaacccactcgagctgtgggctgacagtcccactgggatcgtcccatggagacaattgcaagtcttttgcatgagctaaaccccgctccacatggaaccgaaggtgctcattgtcagctaccacgcaatgccattatcacctttcagcccaagtgccacagaccaacactggctatactccaatgaggtgtggcattcgggttcttctgccttcaggtcacaacctttctgactcagctgggctacattaaacctgaagctctgtacaatgtggagagcggtgttgccttcattacaagtggtgcagcattggattttcaagtaagtctaagtgtttctattgtccttaaaatgacatatgtccagttatttaaaaaaattacaaaatacaaatgcccgtgttaatttagctagtctcagacattacattcgacaacatagaaaagccaaaagatctccagttataagcacaaaactaaggaaagttatggatcagtgacttttgtcactaatccattttcttttttaagtcacctccctttatggccttgcttggctggtttttacattgtgcatgacttgtctgttggaccctggggaggtggggcaggtcctatggtaggatttgtttttggaagaacagcaggttttggcctaagggctggaggcttcagctgcacgcccattctgggtgccaccataggcttgaaagtactcattgtgtcactggaggagctcgtgctacgtcgaatctgaggctcggagctcctgagggcaacgttgtgcaaagggctgagagattccgtggaagtggcaggggtgggagagtttttcacttgctccagggtatccagcaccacatcaggggcatgctttgctgtgctctgtctctccagttctcggagttcattcaaagctgtgttcatcgtttcttcaatatcctgagcaattgtctctgggtccagtggcttgtggtcattgaagcccgtgtattgccctgatgacgtggaccttctaatgggagggctgtcgatcttcttgagggagtcgtgccggctgatgttggtcaggctgccatggccaggcctgcgcctccgctcaggactgtcattgttgaggccacggttctgcagcaggccccgggggtgactggcaaggcttggggaccctaggtcaactgaggagttagaaagggcatgtggagggtggagcgggcaatggccatcactggtcctgccaggacgccttactggagggggtggctctcctctttttcgttgcctggctaaatagccgtcaggatgacggtctgtcggggagttcatgtccttggatgaggacttgtcttccgtgactggcccactgctggcctcactgtcggctttttggctcagagtgtctgaaaacgtatcatccatatcctgcaccactatatactggtgaggcaccagcccgtcaatcccgttgtgcctgccttcccaccagtcctcagatgcacggtgatacagcagcagggaggcacccttcttgaaggatagttctctggcagaccgcccaacatagtcaaacttggctattgcttctattggctcacattcatcttcacttgtgtggggctctgtaccagcatcttggtccacttcctccaatgtaccgtgctcactgtatgggctgtcgcaatagtcatctccagccatacatttctcataaacagggccatccagctctttagcatctgggaaaatagtctcatggtggatgatgatggttttgataatttcattcacatgtgcctggcaagacacttgatcctgtatttctgggacaggcatcaatgttgggccaaagcaaatggccaggttataagggtccatcatattctcatcgctgtactgtgatagatgattgaggaaggcaaagaggtacctcatcactataaggaccgacctgggcaaagtcaggaggagtttgcggatgtgaagcgccctctcatagagattatctattctgatacaagaaatcagatcgttaaatctttccttaggaaagagggggttttccagcccacggaaatagagcttcagaacgccagcaactgagttaatatcatggttactctggtcatcagccaaaggattttcacctctctcaaatgaatttttaatatcattgacttccacctgggaaccagacactctgaaaatcccctgatgctgaagaccatagagattgatgaaccgaatacagctttccacaatgaggggaataacctgtcctgagtccttgacgaatgtttccaaatccccattaaacaacttagtattatactgtgagcggggcctggacttcctgtgtttctggggcttagggggaacatttggaggccttgtagtcatatattcagctctatgaccttctcccagggtcctctgcagcaagtcatgtttggcttgaagttttgtgatgagattactgccttccaaatattctctgagtttcatgaagtagaactgttcagtttcctgctggttggctcttctcttggcgatgctgggtttactcaggtaggtttcagagacagtggacttcactgattctgtggaacgactgtgctggaagcattcagaaacatcatagtcctcgatggtgaccatatcttgtatcgtctgcaaggtggcttcagtcgttttcttaacctcttcattctcgattttgagcgtggcaaggcgggactgcaactgttggtacctgagcatgagctctgcctggactggctgctgggcactgacctggcacacctcatcacccatgtgagactgaaactcaaacttcattggtggacagaacgcagcagggtacatctccatgaatctctgcttatcgctcctgggctctaaattatcaactgcattctcaataatgtctaagccctcatgtctggaggtttcaaggttgtactccgcagacagatatgttcttagggctctgttcagacttgcatggtagccaagatcacagcaatcaattaaatcagaaagatcatgaatatagtacttgaaaactgaggcattggtggcttcaagtgttaggagatattcgttccgtgccttaattgattttagcttattttctgaatattttgcttgtcttttttctttcattttttcaattttctttacagagcttcgccgttgatgtctctcctctagtcgaatatggaagactggatcaccagatctcccaatttgcttttcctcttgtttttcggcctctttcagcttgctctctgcactgatgctctctgcatgatacatatggtatgttttcatcaccgtataaagctcattaagaaccttcattaaatcctcatgaagttggaatgcaatctctttgctctttttaaacatcctggtagaatcctcacttatctgcatgaaccgcataatcacattgttcagatagatgtcactcaaggttgcatggtctttgctttctctccttacttggttcaggagcaaataccagcagttcactggagacaacaggttctggtctttcttgtattgttgatgatccttagtgcttcttgtttttgccatgaacctttctgctaacttctctagattccgggaatattccgtctcaatttcagctttttttcggaagaaatcttgcagatcctggagaagctgaactcgcatctccgtttgctgctccaggcatttttgttgttctaccagttgagctcgaatttctttgacttgactttcatactcggctatgatctctttgtccttcttgaatcggctcggggtggacattatccagctgttccgggtttgctttcaatgggcaagttttgttcagtggtcacaacccgttctccttggagaggcagagttgtactcccacacgcaggcaatccagaggcagcgccg

SEQ ID NO: 11098 - RNA, 2258 nt, Homo sapiens
  source 1..2258: mol_type = other RNA
ctgaatagctgggactacaggtgcacgccaccatgcctggctatttgttgttgttgttgttgttgttgttgttgttgttttgtagaattggggttttgccacgttacccgggctggtcttgaactcttaagctcgagtgatctgcatcttggcctcctgaagtgctgggaatacaggtgtgagccagtgagcccaacccacagtgatttttaagaactgtttctttgtggaaaatgactccttccaaaagttaaatgctccttcatggagctgaagagaaagtgaagagattaagggtagcaatacttcttagccacaaaacatgagtttccctgacttgatctttgacttggctctttactgatccagccaaagctgaagccagggcactgggggagcatgacagccttgccagagagggaggccggcccacccaggaatgcccatccaatcggtccagactgggatttggagcctgtctgtggcctactggctcagtcaccttgggcaagtcatttaacttctctgagccatcagcttttcatttgccaaatgaggatggtgatactatctgccttgcagggttgtcgtgagggttacatgggagagctgtgtgatggctaccatcatcacatcttcatcttcatcatcatcaagtgtttaggcctcacccgggagcaacggggccagtaaaaagctttctgcccggtgtgggaaggttggacttaggagttggacaggccactctagaggtcaatgtggagaggggactggccactccagttgaccttcctgagtagtacccttaggcatgaattggactgacccagcagaagtttggcccaggattgtggccgagaaacaaaatctgaatgtaactaacacagctttaccttatccacttgcctgggatggtacttatgctaatcctattccaagcaaaagcaactcaaactaataaaagctgcgcctccgctctgggttccacaccatctgtcggtccacacgcttgggattagctcttcccatggagcccagactgtctgctcggctgcgtggactatcagaggccagcctggaggcacgggggcggtgccatccattcatgagcacatatgcatggagccctgcatggggccaagccctatgccaaggactggaggtccagtgaaggagagacggacaaggtcgctgctcccaggaagagctctgcagggtggtgaaatatagtagtaacttcatctgactgacatgggggaagtttagaggtgtccttggcatattcacagtgaaatccatcaccctttcaccatgttgggtgatagcaaccgtatggcgcttcctagtgacagccagtgtgcgttctgttaggcagcaccagcgcactgcagctaatgaagcacattcctgcaggcctgtctcctagggctctccgaatcctctgtctgcaaaggaacggcaccatgggaaaatctagcacagccagcatcagccatcacccaaactcaaaagcgtctttgaacggcagagacaggcccattttcctctctgcctggcccagggctggaaccgtcctcaggtcactttttgtgggtctgtacaaacgtgccgactggcagcgagccgctcttcacctgagcccggatttcagctcggtgctttaatgtgaagaccagggctctcaccgtccgccggtacggcccattaatgaggcgggagcagagatgaaacgtttcccgttcaatattttcaaccagtaggtgatccatctttaattccaaggcttctgagagtaatttctgagcatttttcctcaacgactcggttttgggatcacttctaacttcaatagaaggtctatttgaatgtttttcagtgaaagttttccactcagtgtaaacttctctggcaagagaagccacttctgaatctgagtgtttacgcatcttgttcacagtgtgaccttcagagattcaatcgtggcctgcttgtaaacctttcctccagaatctttcttctgagggctattctggattctaggcgttcgaatgacgaatttatccattgttaggggactccgactaccttgacgtgcttgcagcgtgttcaggaaaagcagccctggtagctgctgttggcgccctccagactgcaacctcgtaggctcccaagcccagtcgtctgtgttgaaactaaacagacgcttcctcccagggcggtagttcctctgaagaaactccgccggccctcgcgcctct

SEQ ID NO: 11099 - RNA, 6168 nt, Homo sapiens
  source 1..6168: mol_type = other RNA
ctgaatagctgggactacaggtgcacgccacctcacctggctaattctatattttttttggtagagacaaagtttcaccatgttggccaggatggtctcaaactcctgggcctcatgtgacctgccctcctcagcctcccaaaagtgctgggattacaggcctgagccaccatgcccagccaaaatacatttttacacccattctatctcaaagaataatttaaaggagtaaatattcagctctattttcaccacaatgaagtaatgcttaagcaatcatgtacattattttttcctaataatgtaaccctctagtttcatgccctatgtaactgatctgatctaaaaggatactgtacacgtagcagctcagggaagttgacacaactgttttaagtcgtaagacctagtgtttcagcctgtatgtgattttggacagtcatgtaaccctctctgagcctcagcttccttaactgtaaaatgggtcctactttcttttcaagggcattgtgaagattaagtatgtgagtagatgtaaaaatgctttgtaaatacgtactacccaaacacaaggtattgcactgtattcaaatgtaaataaaatatctatttattcccacagtcaggaaaaatccagttcaactactatgctttaaatcaagttttcttttgaaagctactaagccctgtcttaaatctatcaagaaacaatgaaatttcactttaagttttatgtgtaagcacactcaatatccttaggaaaaatgcctgttacacagataagaagaacatacaggccaaccaacttggttaaaaatgtaatgacttggtggccgggcgcagtggctcacgcctgtaatcccagcactttgggaggccgaggagggcagatcacgaggtcaggagatcgagaccatcctggctaacacggtgaaaccctgtctctactaaaaatacaaaaagattagctgggtgtggtggcgggcacctatagtcccagctacttgggaagctgaggcaggagaatggcatgaacccgggaggcggaggttgtagtgagctgagatagcgccactgcactccagcctggacaacagagcgagactgtctcaaaaaaaaataaaaataaaaaataaaaaaaaaatatatatatatatagtgacttgatactaggactaaattccagaaatccatgtcattgcatgttccttgatctatgaaattaaaatcaccattaagtttaagattagccgggtgtggcagtgtgcgcctgtagtcccagctacttgggaggctgatgtgggagaattgcgtgaacctgggaggtggagcttgcagtgagccgagatcacgccattgcactccagcctgggtgacagagcaagactccgtctccaaaaaaaaaaaaaaaaaagattaaaagattttaagcttaaacatacaaaacagtcagtattaagacaatgtattagaaaggactgaaagttgtaataacccaaaatttgtaaaaggaaacatgagagtcaagatagttgatcttgcattaattacatttagcttataattcaattgacctttcttaaaacgcaaagaaacggtctattaccacatgaaagatatgttttaacacagttggcagttggttcctacttgagagttactacacccataaaagattcatgaagagtattatagccacctcttgaactatttccaaacagtttaatataaatttgttaaccaacaaaagtgcacatattaagtaaatcaaagttcctttgcttttggctggaactgtaacaactcaaagtggtgaggagagacaactttattctgagattagaggttgtttttttttttgttttgttttgttttgtttttgagacaaactctcactctgtcacccaggctggagtataatagcagtcttggctcactgcaaccgccgcctcctggattcaagcgattctcctgtctcagcctcccaagtagctgggttaacaggtgtgcaccaccatgcccagctaattttgtattttaagtagaggcagtgtttcgccatcttggccaggctgacttcgaacgcctgggctcaggtgatctgcccgcctcagcctcccaaagtgctgggattacaggcgtgagccaccacccccagccctgatcagaagttctaattggctcttaatcaaaaatttatttctgagaaccatcttacaacaaaggatcccagacatttaaaatatgggggtggggtggggaggaacactggtttaaaactcaccagtatgttctttagacactagaatcaccacagccaaaagcagggagtatgttttgtttttaaatgaaaaataccctcagtgcagcccactttccgttcttggccctttagatccactttccgttcttggccctttagatacccctcgcaaaaagtgctaaacatatttacagcaatgtgcataagtgagctctgagttaatttcagatctagacaaaaaatctgaggctaagctttatgtcacaacaagttttacaagtccctccacatatcaataacataggcattcacagaaccaaacaacagtaaggaaaggctattacaactggaatacccctgggggttcagttccattagcagtagcaaaggaaaacgatcagataaacctacaaaaacagcagaagcattatgaccaaacctcaggtcattaaatcacgaaagtacagccttacaataggtttcactccattagctctatcctgccaatatgcctgaagatgtcctattggtgatcacagaagaggcgaaaacatacgatttaacttacttaactttttaacagttttttcatttcaataaatttattttgattggttgaattgtttaagaggaagagaagaatatgttcatgtttttcaacttgtttctgtaactctgtgcagcagcaattcatcctatacatcttttctgtatttaaagcactctgcctttgaggtgtgatgttttttgccagaccaaatgtcactagcttatcagctacatcgacagtcccattctcagaacatttctcaactgacactgtatggacattctttgtaattcctttcacagaaagcattacattctgattcaacatgaaattttttaatagcattattattaattgagaagagcttccattcaattccattaatccttcaagtgaacatctaataatttggaaaggaagcgccaggtggctagaggtgattggttgcactctgcaaagaggcagggtttcaatgtttccatagtctgcatagagcacttccacatcagtgtctgatgtccccagaacaactgcacgataccaaaaatcatcacttgtgtatttggcacagcatgcgtctccaattcttggtctatagggtggtcgacttttcggagcattgcagtattctaataattcagctgtcaacatgcacagcttttcctgattttctggcatcccttttggtagagcataaaacaagtttgggcttatgatttctaatacatttgcttgtatagttttatccactggcaattctatcgtcttccattgctcagctgaagaggtagcttgaagtccctgtacatgaacttgaagctcatgtttattaacaagtctgtcatttggtaagtctttatgtggtgaagcagattttaaaaccagatgttcatcaatcagaacatcactaattattctgggataacaagtggagagatcggtgagttcaactcctatcccattttcagtgacttcaaccactctggcttgcaattttatcccagcaacacacatctggaatcttgttatggcttcttcagaccaatgtttgtttctagactgtatatctgcaaaaaaagcacaacaaggttgtcctatctctgccttgaaaccattaggtaacttctgctggcagtgttctgctaatgacttgttcaaatcattgagtttctttaaagcatcctctttaagcacatggcaataaaattctccaggactatatatcacacagaccacaacatctactgtttggtcaacaccaagttcaacccatgtccactccaatggatttacttttccttccacacccaagggaacactggtttctttcacgtcactgggtttatctgtcaccatactctgttctcccacagcaaagcctgcatctaggagaactttgctaacactgacatgaggcgtctcggatttatcaataagctccaccagggaactgttttccaacttgtccaccactttcactgtgattattttgttctgtacaagttttttcatgagacaaatagcttctggagtccaaattcctaatgatggctttactcctgagaactgagcacaacatatatcaccaatggctggataaaaatcagagcgtggaggcaactgatcacagtacttgctaagggatgcctgaagttcagcaagctttcggccactttgcagttgttgacaaaagaagtcttctggtgtttgaatgtgggcaaccacaccacaaaactcatcacctacattcaaagttaacacttttgggattaggtcacttttgtctacgacaatgttgttttcagttgtcatttttccaacatcttcaggatcactttgatctgcattttccttcttagaatcttgtccactgggtttcaagccatatcccatttctataagcacatggtctaaaagttttcctgaatttggcagctcaacttctacagcaaaggtaaccacttcctcttccaagatgtcgacaatctttatggagcagtactgctccattaacagtggtttagtagctttgatacaatcactgctccaattcccttctgctgggataacattggctacaaagcactttatggcacaaggaggaaacaagtcaatgttcctgttgaggtggtaaattctgtttaatggaattatttcttcatttccataatcaatatataagacatgtgccttcttttgctgcacatcaacgttttgtatgattgctctgttccaggtctgatcaacagtgtacttggcaatacaaacttcccccttaacaggaatatagtctttttcatgcacatttgcatatgtttcttttaagctggcagagagttggttcatgtattctaaaacttctgaagaatataactgcacgtagaagtcccctgggtgtttgaattcggtaaccgtaccctttatttccatggttttcttgagttgtagacttctcaaatcagaaaacattattctctcagcccaaatggctatttccttagtaactccaagtggacagtcactcttattgtttacctccacatcctttgtttcaatagatgatttattttcaagtttgtggaaatttggctgaacaggcctgcacacgatgctgtgtgcagaccagtctcttctttgacatgctgtggagcaatagtaggtctgcttgcactgagagcacctcagcgatccaaataggccacagcgatggcaagttgtggaccgaagaggaggtcctaaggaggtgaagagccctggattacttatggacaaggaattctcgaccaacttgtttagtttttttgattttgcaggacgtacattatttccaggcttaatattcacttctttgggtggtgaattactttcagcacttggtggtgacactgagtttcctgctggcaattttttcctgtctcctttggagccaactacttctccgttgatgccattcgggtttgaagaaactgaattgtcttcctgactagccaaatattgtttggtttgctcacaaagcaaaaaattgttctttttatttccattctctgagcttttcagcctgaaattagggtggttaggaagtgttccaggacttcttaaagactcatgtggtggaagcttgttttcatttttctcaaaattaaatggctctgtcatcttacaaggaggtgcttccaaattatttcttgacatcacattaaatggcgatttaacactcatcgaggcctggaaagaggcaagaggaccgcggatccgaacctgtctctgcggtctggcggtgatggcgactgccgatgctgggagccctgccgcctgggatgcgccctgcacttccctcgcctccaatccccagtgc

SEQ ID NO: 11100 - RNA, 6339 nt, Homo sapiens
  source 1..6339: mol_type = other RNA
ctgaatagctgggactacaggtgcacgccacctcacctggctaattctatattttttttggtagagacaaagtttcaccatgttggccaggatggtctcaaactcctgggcctcatgtgacctgccctcctcagcctcccaaaagtgctgggattacaggcctgagccaccatgcccagccaaaatacatttttacacccattctatctcaaagaataatttaaaggagtaaatattcagctctattttcaccacaatgaagtaatgcttaagcaatcatgtacattattttttcctaataatgtaaccctctagtttcatgccctatgtaactgatctgatctaaaaggatactgtacacgtagcagctcagggaagttgacacaactgttttaagtcgtaagacctagtgtttcagcctgtatgtgattttggacagtcatgtaaccctctctgagcctcagcttccttaactgtaaaatgggtcctactttcttttcaagggcattgtgaagattaagtatgtgagtagatgtaaaaatgctttgtaaatacgtactacccaaacacaaggtattgcactgtattcaaatgtaaataaaatatctatttattcccacagtcaggaaaaatccagttcaactactatgctttaaatcaagttttcttttgaaagctactaagccctgtcttaaatctatcaagaaacaatgaaatttcactttaagttttatgtgtaagcacactcaatatccttaggaaaaatgcctgttacacagataagaagaacatacaggccaaccaacttggttaaaaatgtaatgacttggtggccgggcgcagtggctcacgcctgtaatcccagcactttgggaggccgaggagggcagatcacgaggtcaggagatcgagaccatcctggctaacacggtgaaaccctgtctctactaaaaatacaaaaagattagctgggtgtggtggcgggcacctatagtcccagctacttgggaagctgaggcaggagaatggcatgaacccgggaggcggaggttgtagtgagctgagatagcgccactgcactccagcctggacaacagagcgagactgtctcaaaaaaaaataaaaataaaaaataaaaaaaaaatatatatatatatagtgacttgatactaggactaaattccagaaatccatgtcattgcatgttccttgatctatgaaattaaaatcaccattaagtttaagattagccgggtgtggcagtgtgcgcctgtagtcccagctacttgggaggctgatgtgggagaattgcgtgaacctgggaggtggagcttgcagtgagccgagatcacgccattgcactccagcctgggtgacagagcaagactccgtctccaaaaaaaaaaaaaaaaaagattaaaagattttaagcttaaacatacaaaacagtcagtattaagacaatgtattagaaaggactgaaagttgtaataacccaaaatttgtaaaaggaaacatgagagtcaagatagttgatcttgcattaattacatttagcttataattcaattgacctttcttaaaacgcaaagaaacggtctattaccacatgaaagatatgttttaacacagttggcagttggttcctacttgagagttactacacccataaaagattcatgaagagtattatagccacctcttgaactatttccaaacagtttaatataaatttgttaaccaacaaaagtgcacatattaagtaaatcaaagttcctttgcttttggctggaactgtaacaactcaaagtggtgaggagagacaactttattctgagattagaggttgtttttttttttgttttgttttgttttgtttttgagacaaactctcactctgtcacccaggctggagtataatagcagtcttggctcactgcaaccgccgcctcctggattcaagcgattctcctgtctcagcctcccaagtagctgggttaacaggtgtgcaccaccatgcccagctaattttgtattttaagtagaggcagtgtttcgccatcttggccaggctgacttcgaacgcctgggctcaggtgatctgcccgcctcagcctcccaaagtgctgggattacaggcgtgagccaccacccccagccctgatcagaagttctaattggctcttaatcaaaaatttatttctgagaaccatcttacaacaaaggatcccagacatttaaaatatgggggtggggtggggaggaacactggtttaaaactcaccagtatgttctttagacactagaatcaccacagccaaaagcagggagtatgttttgtttttaaatgaaaaataccctcagtgcagcccactttccgttcttggccctttagatccactttccgttcttggccctttagatacccctcgcaaaaagtgctaaacatatttacagcaatgtgcataagtgagctctgagttaatttcagatctagacaaaaaatctgaggctaagctttatgtcacaacaagttttacaagtccctccacatatcaataacataggcattcacagaaccaaacaacagtaaggaaaggctattacaactggaatacccctgggggttcagttccattagcagtagcaaaggaaaacgatcagataaacctacaaaaacagcagaagcattatgaccaaacctcaggtcattaaatcacgaaagtacagccttacaataggtttcactccattagctctatcctgccaatatgcctgaagatgtcctattggtgatcacagaagaggcgaaaacatacgatttaacttacttaactttttaacagttttttcatttcaataaatttattttgattggttgaattgtttaagaggaagagaagaatatgttcatgtttttcaacttgtttctgtaactctgtgcagcagcaattcatcctatacatcttttctgtatttaaagcactctgcctttgaggtgtgatgttttttgccagaccaaatgtcactagcttatcagctacatcgacagtcccattctcagaacatttctcaactgacactgtatggacattctttgtaattcctttcacagaaagcattacattctgattcaacatgaaattttttaatagcattattattaattgagaagagcttccattcaattccattaatccttcaagtgaacatctaataatttggaaaggaagcgccaggtggctagaggtgattggttgcactctgcaaagaggcagggtttcaatgtttccatagtctgcatagagcacttccacatcagtgtctgatgtccccagaacaactgcacgataccaaaaatcatcacttgtgtatttggcacagcatgcgtctccaattcttggtctatagggtggtcgacttttcggagcattgcagtattctaataattcagctgtcaacatgcacagcttttcctgattttctggcatcccttttggtagagcataaaacaagtttgggcttatgatttctaatacatttgcttgtatagttttatccactggcaattctatcgtcttccattgctcagctgaagaggtagcttgaagtccctgtacatgaacttgaagctcatgtttattaacaagtctgtcatttggtaagtctttatgtggtgaagcagattttaaaaccagatgttcatcaatcagaacatcactaattattctgggataacaagtggagagatcggtgagttcaactcctatcccattttcagtgacttcaaccactctggcttgcaattttatcccagcaacacacatctggaatcttgttatggcttcttcagaccaatgtttgtttctagactgtatatctgctaactggcaccgtattccctgaaagggaaggtttaaaaatgttgatgatatcattcggagttcatctgcagtaacttcttcgatgtttccataatccacaaaatgtactttaacatgtccatttggtaagatttccttgactaaagcacgataccaactaccatcacctgcaaaaaaagcacaacaaggttgtcctatctctgccttgaaaccattaggtaacttctgctggcagtgttctgctaatgacttgttcaaatcattgagtttctttaaagcatcctctttaagcacatggcaataaaattctccaggactatatatcacacagaccacaacatctactgtttggtcaacaccaagttcaacccatgtccactccaatggatttacttttccttccacacccaagggaacactggtttctttcacgtcactgggtttatctgtcaccatactctgttctcccacagcaaagcctgcatctaggagaactttgctaacactgacatgaggcgtctcggatttatcaataagctccaccagggaactgttttccaacttgtccaccactttcactgtgattattttgttctgtacaagttttttcatgagacaaatagcttctggagtccaaattcctaatgatggctttactcctgagaactgagcacaacatatatcaccaatggctggataaaaatcagagcgtggaggcaactgatcacagtacttgctaagggatgcctgaagttcagcaagctttcggccactttgcagttgttgacaaaagaagtcttctggtgtttgaatgtgggcaaccacaccacaaaactcatcacctacattcaaagttaacacttttgggattaggtcacttttgtctacgacaatgttgttttcagttgtcatttttccaacatcttcaggatcactttgatctgcattttccttcttagaatcttgtccactgggtttcaagccatatcccatttctataagcacatggtctaaaagttttcctgaatttggcagctcaacttctacagcaaaggtaaccacttcctcttccaagatgtcgacaatctttatggagcagtactgctccattaacagtggtttagtagctttgatacaatcactgctccaattcccttctgctgggataacattggctacaaagcactttatggcacaaggaggaaacaagtcaatgttcctgttgaggtggtaaattctgtttaatggaattatttcttcatttccataatcaatatataagacatgtgccttcttttgctgcacatcaacgttttgtatgattgctctgttccaggtctgatcaacagtgtacttggcaatacaaacttcccccttaacaggaatatagtctttttcatgcacatttgcatatgtttcttttaagctggcagagagttggttcatgtattctaaaacttctgaagaatataactgcacgtagaagtcccctgggtgtttgaattcggtaaccgtaccctttatttccatggttttcttgagttgtagacttctcaaatcagaaaacattattctctcagcccaaatggctatttccttagtaactccaagtggacagtcactcttattgtttacctccacatcctttgtttcaatagatgatttattttcaagtttgtggaaatttggctgaacaggcctgcacacgatgctgtgtgcagaccagtctcttctttgacatgctgtggagcaatagtaggtctgcttgcactgagagcacctcagcgatccaaataggccacagcgatggcaagttgtggaccgaagaggaggtcctaaggaggtgaagagccctggattacttatggacaaggaattctcgaccaacttgtttagtttttttgattttgcaggacgtacattatttccaggcttaatattcacttctttgggtggtgaattactttcagcacttggtggtgacactgagtttcctgctggcaattttttcctgtctcctttggagccaactacttctccgttgatgccattcgggtttgaagaaactgaattgtcttcctgactagccaaatattgtttggtttgctcacaaagcaaaaaattgttctttttatttccattctctgagcttttcagcctgaaattagggtggttaggaagtgttccaggacttcttaaagactcatgtggtggaagcttgttttcatttttctcaaaattaaatggctctgtcatcttacaaggaggtgcttccaaattatttcttgacatcacattaaatggcgatttaacactcatcgaggcctggaaagaggcaagaggaccgcggatccgaacctgtctctgcggtctggcggtgatggcgactgccgatgctgggagccctgccgcctgggatgcgccctgcacttccctcgcctccaatccccagtgc

SEQ ID NO: 11101 - RNA, 6282 nt, Homo sapiens
  source 1..6282: mol_type = other RNA
ctgaatagctgggactacaggtgcacgccacctcacctggctaattctatattttttttggtagagacaaagtttcaccatgttggccaggatggtctcaaactcctgggcctcatgtgacctgccctcctcagcctcccaaaagtgctgggattacaggcctgagccaccatgcccagccaaaatacatttttacacccattctatctcaaagaataatttaaaggagtaaatattcagctctattttcaccacaatgaagtaatgcttaagcaatcatgtacattattttttcctaataatgtaaccctctagtttcatgccctatgtaactgatctgatctaaaaggatactgtacacgtagcagctcagggaagttgacacaactgttttaagtcgtaagacctagtgtttcagcctgtatgtgattttggacagtcatgtaaccctctctgagcctcagcttccttaactgtaaaatgggtcctactttcttttcaagggcattgtgaagattaagtatgtgagtagatgtaaaaatgctttgtaaatacgtactacccaaacacaaggtattgcactgtattcaaatgtaaataaaatatctatttattcccacagtcaggaaaaatccagttcaactactatgctttaaatcaagttttcttttgaaagctactaagccctgtcttaaatctatcaagaaacaatgaaatttcactttaagttttatgtgtaagcacactcaatatccttaggaaaaatgcctgttacacagataagaagaacatacaggccaaccaacttggttaaaaatgtaatgacttggtggccgggcgcagtggctcacgcctgtaatcccagcactttgggaggccgaggagggcagatcacgaggtcaggagatcgagaccatcctggctaacacggtgaaaccctgtctctactaaaaatacaaaaagattagctgggtgtggtggcgggcacctatagtcccagctacttgggaagctgaggcaggagaatggcatgaacccgggaggcggaggttgtagtgagctgagatagcgccactgcactccagcctggacaacagagcgagactgtctcaaaaaaaaataaaaataaaaaataaaaaaaaaatatatatatatatagtgacttgatactaggactaaattccagaaatccatgtcattgcatgttccttgatctatgaaattaaaatcaccattaagtttaagattagccgggtgtggcagtgtgcgcctgtagtcccagctacttgggaggctgatgtgggagaattgcgtgaacctgggaggtggagcttgcagtgagccgagatcacgccattgcactccagcctgggtgacagagcaagactccgtctccaaaaaaaaaaaaaaaaaagattaaaagattttaagcttaaacatacaaaacagtcagtattaagacaatgtattagaaaggactgaaagttgtaataacccaaaatttgtaaaaggaaacatgagagtcaagatagttgatcttgcattaattacatttagcttataattcaattgacctttcttaaaacgcaaagaaacggtctattaccacatgaaagatatgttttaacacagttggcagttggttcctacttgagagttactacacccataaaagattcatgaagagtattatagccacctcttgaactatttccaaacagtttaatataaatttgttaaccaacaaaagtgcacatattaagtaaatcaaagttcctttgcttttggctggaactgtaacaactcaaagtggtgaggagagacaactttattctgagattagaggttgtttttttttttgttttgttttgttttgtttttgagacaaactctcactctgtcacccaggctggagtataatagcagtcttggctcactgcaaccgccgcctcctggattcaagcgattctcctgtctcagcctcccaagtagctgggttaacaggtgtgcaccaccatgcccagctaattttgtattttaagtagaggcagtgtttcgccatcttggccaggctgacttcgaacgcctgggctcaggtgatctgcccgcctcagcctcccaaagtgctgggattacaggcgtgagccaccacccccagccctgatcagaagttctaattggctcttaatcaaaaatttatttctgagaaccatcttacaacaaaggatcccagacatttaaaatatgggggtggggtggggaggaacactggtttaaaactcaccagtatgttctttagacactagaatcaccacagccaaaagcagggagtatgttttgtttttaaatgaaaaataccctcagtgcagcccactttccgttcttggccctttagatccactttccgttcttggccctttagatacccctcgcaaaaagtgctaaacatatttacagcaatgtgcataagtgagctctgagttaatttcagatctagacaaaaaatctgaggctaagctttatgtcacaacaagttttacaagtccctccacatatcaataacataggcattcacagaaccaaacaacagtaaggaaaggctattacaactggaatacccctgggggttcagttccattagcagtagcaaaggaaaacgatcagataaacctacaaaaacagcagaagcattatgaccaaacctcaggtcattaaatcacgaaagtacagccttacaataggtttcactccattagctctatcctgccaatatgcctgaagatgtcctattggtgatcacagaagaggcgaaaacatacgatttaacttacttaactttttaacagttttttcatttcaataaatttattttgattggttgaattgtttaagaggaagagaagaatatgttcatgtttttcaacttgtttctgtaactctgtgcagcagcaattcatcctatacatcttttcttcaagtgaacatctaataatttggaaaggaagcgccaggtggctagaggtgattggttgcactctgcaaagaggcagggtttcaatgtttccatagtctgcatagagcacttccacatcagtgtctgatgtccccagaacaactgcacgataccaaaaatcatcacttgtgtatttggcacagcatgcgtctccaattcttggtctatagggtggtcgacttttcggagcattgcagtattctaataattcagctgtcaacatgcacagcttttcctgattttctggcatcccttttggtagagcataaaacaagtttgggcttatgatttctaatacatttgcttgtatagttttatccactggcaattctatcgtcttccattgctcagctgaagaggtagcttgaagtccctgtacatgaacttgaagctcatgtttattaacaagtctgtcatttggtaagtctttatgtggtgaagcagattttaaaaccagatgttcatcaatcagaacatcactaattattctgggataacaagtggagagatcggtgagttcaactcctatcccattttcagtgacttcaaccactctggcttgcaattttatcccagcaacacacatctggaatcttgttatggcttcttcagaccaatgtttgtttctagactgtatatctgctaactggcaccgtattccctgaaagggaaggtttaaaaatgttgatgatatcattcggagttcatctgcagtaacttcttcgatgtttccataatccacaaaatgtactttaacatgtccatttggtaagatttccttgactaaagcacgataccaactaccatcacctgcaaaaaaagcacaacaaggttgtcctatctctgccttgaaaccattaggtaacttctgctggcagtgttctgctaatgacttgttcaaatcattgagtttctttaaagcatcctctttaagcacatggcaataaaattctccaggactatatatcacacagaccacaacatctactgtttggtcaacaccaagttcaacccatgtccactccaatggatttacttttccttccacacccaagggaacactggtttctttcacgtcactgggtttatctgtcaccatactctgttctcccacagcaaagcctgcatctaggagaactttgctaacactgacatgaggcgtctcggatttatcaataagctccaccagggaactgttttccaacttgtccaccactttcactgtgattattttgttctgtacaagttttttcatgagacaaatagcttctggagtccaaattcctaatgatggctttactcctgctagtacacactttatagcttgcattggcaattccaacaactttgggattatgggacaaagtctcatcaaactaaggatttcaaagtttccataatctacatatccgaccagtacagattcttcagaagcgtaagccaaaacagaggcacggtaccactgatcatcctctgagaactgagcacaacatatatcaccaatggctggataaaaatcagagcgtggaggcaactgatcacagtacttgctaagggatgcctgaagttcagcaagctttcggccactttgcagttgttgacaaaagaagtcttctggtgtttgaatgtgggcaaccacaccacaaaactcatcacctacattcaaagttaacacttttgggattaggtcacttttgtctacgacaatgttgttttcagttgtcatttttccaacatcttcaggatcactttgatctgcattttccttcttagaatcttgtccactgggtttcaagccatatcccatttctataagcacatggtctaaaagttttcctgaatttggcagctcaacttctacagcaaaggtaaccacttcctcttccaagatgtcgacaatctttatggagcagtactgctccattaacagtggtttagtagctttgatacaatcactgctccaattcccttctgctgggataacattggctacaaagcactttatggcacaaggaggaaacaagtcaatgttcctgttgaggtggtaaattctgtttaatggaattatttcttcatttccataatcaatatataagacatgtgccttcttttgctgcacatcaacgttttgtatgattgctctgttccaggtctgatcaacagtgtacttggcaatacaaacttcccccttaacaggaatatagtctttttcatgcacatttgcatatgtttcttttaagctggcagagagttggttcatgtattctaaaacttctgaagaatataactgcacgtagaagtcccctgggtgtttgaattcggtaaccgtaccctttatttccatggttttcttgagttgtagacttctcaaatcagaaaacattattctctcagcccaaatggctatttccttagtaactccaagtggacagtcactcttattgtttacctccacatcctttgtttcaatagatgatttattttcaagtttgtggaaatttggctgaacaggcctgcacacgatgctgtgtgcagaccagtctcttctttgacatgctgtggagcaatagtaggtctgcttgcactgagagcacctcagcgatccaaataggccacagcgatggcaagttgtggaccgaagaggaggtcctaaggaggtgaagagccctggattacttatggacaaggaattctcgaccaacttgtttagtttttttgattttgcaggacgtacattatttccaggcttaatattcacttctttgggtggtgaattactttcagcacttggtggtgacactgagtttcctgctggcaattttttcctgtctcctttggagccaactacttctccgttgatgccattcgggtttgaagaaactgaattgtcttcctgactagccaaatattgtttggtttgctcacaaagcaaaaaattgttctttttatttccattctctgagcttttcagcctgaaattagggtggttaggaagtgttccaggacttcttaaagactcatgtggtggaagcttgttttcatttttctcaaaattaaatggctctgtcatcttacaaggaggtgcttccaaattatttcttgacatcacattaaatggcgatttaacactcatcgaggcctggaaagaggcaagaggaccgcggatccgaacctgtctctgcggtctggcggtgatggcgactgccgatgctgggagccctgccgcctgggatgcgccctgcacttccctcgcctccaatccccagtgc

SEQ ID NO: 11102 - RNA, 6138 nt, Homo sapiens
  source 1..6138: mol_type = other RNA
ctgaatagctgggactacaggtgcacgccacctcacctggctaattctatattttttttggtagagacaaagtttcaccatgttggccaggatggtctcaaactcctgggcctcatgtgacctgccctcctcagcctcccaaaagtgctgggattacaggcctgagccaccatgcccagccaaaatacatttttacacccattctatctcaaagaataatttaaaggagtaaatattcagctctattttcaccacaatgaagtaatgcttaagcaatcatgtacattattttttcctaataatgtaaccctctagtttcatgccctatgtaactgatctgatctaaaaggatactgtacacgtagcagctcagggaagttgacacaactgttttaagtcgtaagacctagtgtttcagcctgtatgtgattttggacagtcatgtaaccctctctgagcctcagcttccttaactgtaaaatgggtcctactttcttttcaagggcattgtgaagattaagtatgtgagtagatgtaaaaatgctttgtaaatacgtactacccaaacacaaggtattgcactgtattcaaatgtaaataaaatatctatttattcccacagtcaggaaaaatccagttcaactactatgctttaaatcaagttttcttttgaaagctactaagccctgtcttaaatctatcaagaaacaatgaaatttcactttaagttttatgtgtaagcacactcaatatccttaggaaaaatgcctgttacacagataagaagaacatacaggccaaccaacttggttaaaaatgtaatgacttggtggccgggcgcagtggctcacgcctgtaatcccagcactttgggaggccgaggagggcagatcacgaggtcaggagatcgagaccatcctggctaacacggtgaaaccctgtctctactaaaaatacaaaaagattagctgggtgtggtggcgggcacctatagtcccagctacttgggaagctgaggcaggagaatggcatgaacccgggaggcggaggttgtagtgagctgagatagcgccactgcactccagcctggacaacagagcgagactgtctcaaaaaaaaataaaaataaaaaataaaaaaaaaatatatatatatatagtgacttgatactaggactaaattccagaaatccatgtcattgcatgttccttgatctatgaaattaaaatcaccattaagtttaagattagccgggtgtggcagtgtgcgcctgtagtcccagctacttgggaggctgatgtgggagaattgcgtgaacctgggaggtggagcttgcagtgagccgagatcacgccattgcactccagcctgggtgacagagcaagactccgtctccaaaaaaaaaaaaaaaaaagattaaaagattttaagcttaaacatacaaaacagtcagtattaagacaatgtattagaaaggactgaaagttgtaataacccaaaatttgtaaaaggaaacatgagagtcaagatagttgatcttgcattaattacatttagcttataattcaattgacctttcttaaaacgcaaagaaacggtctattaccacatgaaagatatgttttaacacagttggcagttggttcctacttgagagttactacacccataaaagattcatgaagagtattatagccacctcttgaactatttccaaacagtttaatataaatttgttaaccaacaaaagtgcacatattaagtaaatcaaagttcctttgcttttggctggaactgtaacaactcaaagtggtgaggagagacaactttattctgagattagaggttgtttttttttttgttttgttttgttttgtttttgagacaaactctcactctgtcacccaggctggagtataatagcagtcttggctcactgcaaccgccgcctcctggattcaagcgattctcctgtctcagcctcccaagtagctgggttaacaggtgtgcaccaccatgcccagctaattttgtattttaagtagaggcagtgtttcgccatcttggccaggctgacttcgaacgcctgggctcaggtgatctgcccgcctcagcctcccaaagtgctgggattacaggcgtgagccaccacccccagccctgatcagaagttctaattggctcttaatcaaaaatttatttctgagaaccatcttacaacaaaggatcccagacatttaaaatatgggggtggggtggggaggaacactggtttaaaactcaccagtatgttctttagacactagaatcaccacagccaaaagcagggagtatgttttgtttttaaatgaaaaataccctcagtgcagcccactttccgttcttggccctttagatccactttccgttcttggccctttagatacccctcgcaaaaagtgctaaacatatttacagcaatgtgcataagtgagctctgagttaatttcagatctagacaaaaaatctgaggctaagctttatgtcacaacaagttttacaagtccctccacatatcaataacataggcattcacagaaccaaacaacagtaaggaaaggctattacaactggaatacccctgggggttcagttccattagcagtagcaaaggaaaacgatcagataaacctacaaaaacagcagaagcattatgaccaaacctcaggtcattaaatcacgaaagtacagccttacaataggtttcactccattagctctatcctgccaatatgcctgaagatgtcctattggtgatcacagaagaggcgaaaacatacgatttaacttacttaactttttaacagttttttcatttcaataaatttattttgattggttgaattgtttaagaggaagagaagaatatgttcatgtttttcaacttgtttctgtaactctgtgcagcagcaattcatcctatacatcttttcttcaagtgaacatctaataatttggaaaggaagcgccaggtggctagaggtgattggttgcactctgcaaagaggcagggtttcaatgtttccatagtctgcatagagcacttccacatcagtgtctgatgtccccagaacaactgcacgataccaaaaatcatcacttgtgtatttggcacagcatgcgtctccaattcttggtctatagggtggtcgacttttcggagcattgcagtattctaataattcagctgtcaacatgcacagcttttcctgattttctggcatcccttttggtagagcataaaacaagtttgggcttatgatttctaatacatttgcttgtatagttttatccactggcaattctatcgtcttccattgctcagctgaagaggtagcttgaagtccctgtacatgaacttgaagctcatgtttattaacaagtctgtcatttggtaagtctttatgtggtgaagcagattttaaaaccagatgttcatcaatcagaacatcactaattattctgggataacaagtggagagatcggtgagttcaactcctatcccattttcagtgacttcaaccactctggcttgcaattttatcccagcaacacacatctggaatcttgttatggcttcttcagaccaatgtttgtttctagactgtatatctgctaactggcaccgtattccctgaaagggaaggtttaaaaatgttgatgatatcattcggagttcatctgcagtaacttcttcgatgtttccataatccacaaaatgtactttaacatgtccatttggtaagatttccttgactaaagcacgataccaactaccatcacctgcaaaaaaagcacaacaaggttgtcctatctctgccttgaaaccattaggtaacttctgctggcagtgttctgctaatgacttgttcaaatcattgagtttctttaaagcatcctctttaagcacatggcaataaaattctccaggactatatatcacacagaccacaacatctactgtttggtcaacaccaagttcaacccatgtccactccaatggatttacttttccttccacacccaagggaacactggtttctttcacgtcactgggtttatctgtcaccatactctgttctcccacagcaaagcctgcatctaggagaactttgctaacactgacatgaggcgtctcggatttatcaataagctccaccagggaactgttttccaacttgtccaccactttcactgtgattattttgttctgtacaagttttttcatgagacaaatagcttctggagtccaaattcctaatgatggctttactcctgctagtacacactttatagcttgcattggcaattccaacaactttgggattatgggacaaagtctcatcaaactaaggatttcaaagtttccataatctacatatccgaccagtacagattcttcagaagcgtaagccaaaacagaggcacggtaccactgatcatcctctgagaactgagcacaacatatatcaccaatggctggataaaaatcagagcgtggaggcaactgatcacagtacttgctaagggatgcctgaagttcagcaagctttcggccactttgcagttgttgacaaaagaagtcttctggtgtttgaatgtgggcaaccacaccacaaaactcatcacctacattcaaagttaacacttttgggattaggtcacttttgtctacgacaatgttgttttcagttgtcatttttccaacatcttcaggatcactttgatctgcattttccttcttagaatcttgtccactgggtttcaagccatatcccatttctataagcacatggtctaaaagttttcctgaatttggcagctcaacttctacagcaaaggtaaccacttcctcttccaagatgtcgacaatctttatggagcagtactgctccattaacagtggtttagtagctttgatacaatcactgctccaattcccttctgctgggataacattggctacaaagcactttatggcctgatcaacagtgtacttggcaatacaaacttcccccttaacaggaatatagtctttttcatgcacatttgcatatgtttcttttaagctggcagagagttggttcatgtattctaaaacttctgaagaatataactgcacgtagaagtcccctgggtgtttgaattcggtaaccgtaccctttatttccatggttttcttgagttgtagacttctcaaatcagaaaacattattctctcagcccaaatggctatttccttagtaactccaagtggacagtcactcttattgtttacctccacatcctttgtttcaatagatgatttattttcaagtttgtggaaatttggctgaacaggcctgcacacgatgctgtgtgcagaccagtctcttctttgacatgctgtggagcaatagtaggtctgcttgcactgagagcacctcagcgatccaaataggccacagcgatggcaagttgtggaccgaagaggaggtcctaaggaggtgaagagccctggattacttatggacaaggaattctcgaccaacttgtttagtttttttgattttgcaggacgtacattatttccaggcttaatattcacttctttgggtggtgaattactttcagcacttggtggtgacactgagtttcctgctggcaattttttcctgtctcctttggagccaactacttctccgttgatgccattcgggtttgaagaaactgaattgtcttcctgactagccaaatattgtttggtttgctcacaaagcaaaaaattgttctttttatttccattctctgagcttttcagcctgaaattagggtggttaggaagtgttccaggacttcttaaagactcatgtggtggaagcttgttttcatttttctcaaaattaaatggctctgtcatcttacaaggaggtgcttccaaattatttcttgacatcacattaaatggcgatttaacactcatcgaggcctggaaagaggcaagaggaccgcggatccgaacctgtctctgcggtctggcggtgatggcgactgccgatgctgggagccctgccgcctgggatgcgccctgcacttccctcgcctccaatccccagtgc

SEQ ID NO: 11103 - RNA, 2752 nt, Homo sapiens
  source 1..2752: mol_type = other RNA
ctgaatagctgggactacaggtgcacgccactgcacccagctaattttcgtatttttagtagagacagggtttcaccgtgttggccaggctggtctcaaactcctgaccgcaggtgatccgcccgccttggcctcccaaagtgctgagattaaaggcatgaggattatcatattctaaatggcaatagagcactaagactataaataagtctcagtagtaaaaactaaacctaaaagaaaaatgtatccaatgtgacacattttcaatatttacagagcatcctaaatatggaatttaaaaaattacacaaggtagaagcaaacaatctatgaaaatattaaaaattactattataactgattatatcattaagtgcaaactcaaaagaactcaagtatttgttgtaggaaaagaaagtatacctttcatatacttctgattcacccagtatgaaaactagtcatattttaaagaaataaataattttattttttgagatggagtttcgcttttgttgcccaggctgaagtgcaatggcgagatctccggctcagcgtaacctccgcctcctggggttcaagcaattctcctgcctcagcctcccgagtagctgggattacaggcatgtgccaccacacctagctaattttgtatttttcgtaaagatggggtttctccatgttggtcagggtggtcttgaactcccaacctcaggtgatctgcccgcctcagcctcccaaagtgctgggattacaggcgtgagccaccatgcctggcttaaagagataaataattaagggatccttagaagaaatggaacagtttgtaagaaagataaatttcagactttttgctaggagggaaaactattagggctacatactctataattctagaaccatttccttcagaatgcttctgggtgaccttttcaaattaaatttttaaaaatacagtaaaagatagcagtgtcagttgtttgtgggtgaaaatataaacccaacactggatataatacagatcagaaaattttattattgagattacttaaggttgtaaaaaaaaaaaaaaatttaccttttgcctgttctcatactgacatgtcaccactccatttctaaggattccaagtcaattaatgcagaacttttaaaagtattaatgatctctactgtaccaaactgtgcatgctatagttcatcaatcttactcttccaataaacctagagatttaaataagataaaaatgacagcagtctccataatcttaaaatctaggtgaaacaaatgtccttatggtccaataatgtgtataataaaatgtaaccaggtcaccagaccaacatactagtgtgtaactttaataatttctagcagcaaaacacctgaaatagccaataacaaatgttttcattggattgtacattcatttctttgtgagaaataattttaaaaagtactctaaagtattgttcaactgcaggcaaacatgaaagatatcaaagatcttgcttttctccatctttcccaatggaatcaggtgcaactggaaccttattagtttcaacaaaaacagattcaaaggcagcttcctgttcatccaaagaatcagcaaccgtggctcctttagttagtgttgggttggtaaaagattgttgctgcttggaaactttacttgattccaccgttttcctaccttttcttttgccaagaattttgacataattcgcaggtataagtcctgttgtttggccatcaaggctagccagaagccaaccacgcactttgggttgttgttctttgagagctaagttcagcatatcaccagcccggaaagaaatttcttcttcagatacggcagcaaaatcatattctgctctggcaactacatggtcatcctcaccacttgcccagttgatgctgtctgttacttcatcactgtgagtagacaatagtttccaaatgaggtaaggaccaccaaggataacagcaaagaacaagaatattggccaagattttgctgaggtagctgctcggtcctcagcaccaaggcatgccacagttccttcactctctgcccagaggtcttcattctcagagcctcttcttaaacctaacatccgctgtagccgtctgtaaagataccgtatagtcctaaccaatgcaaaagctgaaaacacttttgtaaagtgtattttcaatcgggaaaagtgatttgctacatccaatacagccctgaaactgttatagacagctgaaaaggtagcatccatcatcatactgacagaggcaaatgcatgcacaatactttcaatggactgaaatgcacccctgctgctttcttcagcttgctgaacaaatctactgggtggaagatcatctacacggaggcggttgtagcccagcccattatatccataactataaggactatagcctccataaaatgaatttccataggcaccatatccagaagaaaatgaactgtaagcaggtctaaaagtgttcacactgctacttcctgtctgctgtgatggccttggaagaataggtgggggcactctggtaagtgctggttgtccaggtcttgtcattaaagtaggacccaaatcagcagattggaaagtggggcccggtcctggtcccggtccggctcccggaattcggcgggtctcccagggtttggggggaggtggcggctgggacgccatctcctccgcctcctctcggctcccgctcctacccctgact

SEQ ID NO: 11104 - RNA, 1884 nt, Homo sapiens
  source 1..1884: mol_type = other RNA
ctgaatagctgggactacaggtgcacgccatcatgccgagctagtttttctatttttagtagagacagggtttcaccgtgttgaacaggctggtcttgaacttttgacctctgatgattgccagcttggcctctcaaagtgctaggattacaggcgtgtgccactgcacctggcttcagcatcctaaagtgtcaacattgcccaagttaatatatacatttaatgcacttctggctgtgttcccaatgctctgaaagggttagcaaaacctcttttcttttttcacaggaaaatgataataattcaccttctctagtactatttcctttaaatcatgataatgatgtaatgtcagtgtttgccaggaaacactacttttaataaaaatgaccctatttggttaactgcatctagaggaccatggctacaataagggaatactatagtgtgtttatcttcacttacaattttaatatctaattttatggtattattacttccccaaataaaatctaaagtcattttgtttctatgtctaggtatactatacaatatgcagaaagccattcagctgtctgtctctatacttactaattcattgataagaagtccaatataagagtagtttttattattttagtacaagcataagcaataatttagtttgttttaatatatttttgagaatatattaagttgcaaattgaaactattatattaattttctttgaaataaagtagaaattacaacaatatcagaagctatctttgcaagctttgagaccataagagtgagaagtggaaaagtggaagttggacatacatttagggtaacaatgctgccttattcgcatctggggtattccactatcccttcccgacacactgcttgaaatgatagaattgatgtatttgcattatatcccaatttacacataaattcaatggtatcccctgtttttgcataatattttctgtcacttcttccttttaactttatgttatttttattcatgttttcttcagttattatacatggatgtatgcatcttggtggttccgaccactctccattactacatgttacataattagaaccctgaagttcatagtagggctggcattggtactcgactcttgactgtggcacatacacttttagtagaaaggaggtggtatcaccattgctaataggtggaggaggcccacacttttctgaagaattaatgcaaattggttgtgctgaccatccattttgcaaacatgtaattgatcctgaagaatttccatctgctgttgcatatcctggtttacatttatattgtatttctttatttaaaatataaatagaggaagattcggaaatgaatccattttcaatttctatatctgattttgagcatgttctgacacggatgcatctgggagtaggagaccagcctttctccgtacatgtaactgtggtctgcgcttttggaagaccgtagccaggatggcaggcaacttctgtagagttaccctgtacaaactttcttccataattttgattatatccattttccaaataaggaaaataacattttctgagacatggtactgctggtgaccacccattttgtgtgcaatgaatgtaatcccagtaacttcctgaaggagtctcaaaatgttcatcacagtaataggagtaatattttcctacagctactggaaagtatggtctacgcatattctcatgaaatagacctccatgtttaatgtctggaaaatcacaaggtttcacttgtccattagcacaggaaacccacaaggtcagaatgacattgattagtaacaacatgttagatattctcagtagtatgctaatacaaaagtttcagttgcact

SEQ ID NO: 11105 - RNA, 1701 nt, Homo sapiens
  source 1..1701: mol_type = other RNA
ctgaatagctgggactacaggtgcacgccatcatgccgagctagtttttctatttttagtagagacagggtttcaccgtgttgaacaggctggtcttgaacttttgacctctgatgattgccagcttggcctctcaaagtgctaggattacaggcgtgtgccactgcacctggcttcagcatcctaaagtgtcaacattgcccaagttaatatatacatttaatgcacttctggctgtgttcccaatgctctgaaagggttagcaaaacctcttttcttttttcacaggaaaatgataataattcaccttctctagtactatttcctttaaatcatgataatgatgtaatgtcagtgtttgccaggaaacactacttttaataaaaatgaccctatttggttaactgcatctagaggaccatggctacaataagggaatactatagtgtgtttatcttcacttacaattttaatatctaattttatggtattattacttccccaaataaaatctaaagtcattttgtttctatgtctaggtatactatacaatatgcagaaagccattcagctgtctgtctctatacttactaattcattgataagaagtccaatataagagtagtttttattattttagtacaagcataagcaataatttagtttgttttaatatatttttgagaatatattaagttgcaaattgaaactattatattaattttctttgaaataaagtagaaattacaacaatatcagaagctatctttgcaagctttgagaccataagagtgagaagtggaaaagtggaagttggacatacatttagggtaacaatgctgccttattcgcatctggggtattccactatcccttcccgacacactgcttgaaatgatagaattgatgtatttgcattatatcccaatttacacataaattcaatggtatcccctgtttttgcataatattttctgtcacttcttccttttaactttatgttatttttattcatgttttcttcagttattatacatggatgtatgcatcttggtggttccgaccactctccattactacatgttacataattagaaccctgaagttcatagtagggctggcattggtactcgactcttgactgtggcacatacacttttagtagaaaggaggtggtatcaccattgctaataggtggaggaggcccacacttttctgaagaattgacacggatgcatctgggagtaggagaccagcctttctccgtacatgtaactgtggtctgcgcttttggaagaccgtagccaggatggcaggcaacttctgtagagttaccctgtacaaactttcttccataattttgattatatccattttccaaataaggaaaataacattttctgagacatggtactgctggtgaccacccattttgtgtgcaatgaatgtaatcccagtaacttcctgaaggagtctcaaaatgttcatcacagtaataggagtaatattttcctacagctactggaaagtatggtctacgcatattctcatgaaatagacctccatgtttaatgtctggaaaatcacaaggtttcacttgtccattagcacaggaaacccacaaggtcagaatgacattgattagtaacaacatgttagatattctcagtagtatgctaatacaaaagtttcagttgcact

SEQ ID NO: 11106 - RNA, 4793 nt, Homo sapiens
  source 1..4793: mol_type = other RNA
ctgaatagctgggactacaggtgcacgtcaccatgcccggctaatttttgtatttttattagagacggggtttcaccatgttggccaggatggtctcgatctcttgacctcgtgatccccccgcctcggcctcccaaagcgctgggattacagggggagccaccgcgcccggcctttcttcagtgcaatttctaaagagaaacttaaatcctgttgtattctttcaacacaagcaatgatacttctcagagtctgctcaaaagctcagctctgtggactccgtgacaaaatgtacgcgtccactgccgaccctcttggtttctgaaaccaacctttcttcctgctctcctctttaagagcaaaccccaacatgtataaggtcacagcaagtggtagccaggaaaagctgtgggacccctcatttgagtcacatccatatggcatggagaaagaaaacctctctgccagaaggaactgaactctggaagtcctaaggaaggtcaccatgatcagcagataggaaagcattgccaagggctgtccctcaagagcttagttttcttagggagaccagaaagacatcagatcctgactgccctgttttgctcaagttctgaaatgagtggcatgatgaagagctggtggagctgagggaaagagtcaaccatgtggggtggggtagtgaggaaggtgtatgaggaaacaaactgggccctgacgaaacaggcggattggggaaggagaaagaaggaagggagagaaacctaaccaaagaaacatgggaagctggaaagtcgagggcacagccggaataaaggcacagatgggcaccccacaggaggggccttggccaggttgggatgcagagaaaaacaggcaggagggtgtcaatctatagcatcctgaaccccaaaaggtctgtaactggattctctaagccttgagaagttcacaccaaagcttcagaccagggaaaatattttggaaagatcagtctttccaagagtgagctcctttccaagaagctggacaggaaacccaataaatgtggatctgaaaaaacaaaatccaagagagaagcaaaatgggctgggggtgtgcaataagagaagcaaggaaaatggaaagactgtagctgaggatcttttattaaaaaaaaatggatgggactttggtgatgagagagaaaaagggcaaaagtctgcagttaggaatttaggtgaccgaagactgtcctagacagttgggagggacaggctgatggacagaagagagaaattcctttcaatgacaaccaagctgaactattcgataccagcagaactgggttctttagggattaagccaagacaaagacttgggaatcactcactccgaggatgaagaatgggttaatggctgaggagacagtcaaaggaatagagaggcctggctttgagggcctcttcaccaccagcacaagataaggcaaaggaccatttgtcagagacaccaagaaaggggaatttccatttggatggtcaatagtgtccagttctgccaaggacaagactaagctttgagaaaaagccatggatttggtgattggataactggtaacctttagaaaagtttagttgacagacagagaccgaagtgagttagtaaaagtcatgaagagaatgaatggcaacttaagggaagcaacatactggagaagttgagcagcgggatgaataacaaataggacagatgggaacagaaaaatctgggtgcatacgaaggtggatggaaaggagctggtacagatgggcacaaccagaaaacatgaggaggggaaaggaagggaaaaggaaggcaggcagggagagagacgtgaaatagccacagtcttaggggatgctagagaagcctagaagattcctcaggttggtgcaaagtattataagactaacgcatcagtacagagaatgacccaagaagggtaggagttcattccttaccttcataaagtaggctatccgccaagaatgaaaatgtcaactcaaagctatgggctgttttaagcaaggtggaagataatataagaagcatggtcctttcttcagacttactgccttgacagcacagaattcatcttatttccctcatctcccaagttatttgtatttccctgagatcagctcagaaacaactctctttaggctctctacaatgcggtagagcatgattagaaaagataaaccttcaaacaatagtgttgtccaagacactaccctcacttatcccaggggaacccacggaatttcttcatttgtattaactcctgacatggcatggaagaagaatttttatcaaatacccttggcatcttatatcagattaaaggaccattaaatacactgaggtaaaattggcagagagtatagtttctattaataaatctaagtctattttgtctgttttaggcaacaaaggcaaaatggactttgtgggaaatgtatctcataaaagccctttggaaaaactgcagaccaaaaccaaaaccctccttcatgttttctcgcatgaaacataaacttgccctatttcaaaaagttcctactgagtatgattgtgtgaaagatcacactacttcaaatcatatttattttaaaaatctgtgatgggacagtggcctcactgccaggaagcccaagttctgttttatgctcggtacaactaagtggaagttgattcactttgtctcaagctacataaaataatcagaaaatcaagaagatctcatgctagacaggttagacttgcacccaaaaaagcatctttttttttaacctgctgttttggtttgctgctgaagtctttgaagagaattatgtattcaaagtagctctttgcccattggcatttccccatcttctatgtcttctgtagggcacatcccccccaaagtaagaggccttagtagaaaagcacttccacctgcagttttcccctaggtctgcagagagaaacagtgcagagtgcaatgccacagtcaaggaccaactttcctacagagcccgggccccagggagggtggtcagcagcgcagcctgcccaggctgggatctccctttggtcatagccgtgtttccatatacccctccactcaccctcagaggaggaacggatggaagccaccagcataaataaagggaacacagaagaacaatgtcaccaaagtgcaggtgcaaagcccaaagcagccccctacctctgccagcccagacccgccactaaattctagaggagggtgtctctcaggtcacagtacttttttcttcatttcttttgatttagaaacaaatcagcagggaggacaaggttctcaaggacaaaaaaatcaaagctgaaacgagagcagcacaatccattggtgacgttcatctttttccagaggaatataccattctgttaggacttaggggaaaaaagatcttctggtccaaacgttggtagtcactggcctttggccgccgggtgactttagatctttttccttccaggacaaaagcaatgatcttccgcttgttgtgatgagcgatatagaggacagccacaagaatggctgcagtcaccagatatgcaaagaagtggctgctctccgcgctgccatttccagaaccgttcggataaaggtcatccttctcgctacccgtggaatccgaaagtgtcccttcacggttctcactggaggcagaaccggacatcttttctttctcttctttgggcggtgagccctcctcgggtcctgtatcatcatcttcagcctctttgggctccacatcctcagtaggctctgaagacttaacttcctcctgcgggggagaaatgaggtcagtttcctccccagattcggttttgaaagcatgaggagaaagcttccctttgtcagcaagctggtttgtgtcagccttggggagctccttgttatcagaagggttggagatgggcttggaatggtctttccgggaaggctgctctggaaccaccttgttagggctgtcttttgaggtctgctcctccgcacccgacttgctgggcccgtctattgggccctgctcctctgcaccggacttgttagagccgtcttttggagtctgcttctccgcacccgacttgttagggacgtcttttggggtctgatcctccgcacccgacttgctggagccgtcttttggggtctggccgtccgcacccgacttattagggacatcttttgtggtctgcgcctccgaacctgacttgctagggctgtctttttgggtctttgcctccgcacccgacctgttggggctgtcttctggggtctgcgcctccgcacccgatttgccagtgctgtcttttggagtctgcagctccggatgcgacttactagtgctgtcttttgtggtctgcgcctccgaacccgacttgctagtgctgcctttttgggtctttgcctccgcacccgacttgttggagctgtctttttgggtctttgcctccgcacccgacttgttgggggtgtcttctggggtctgcgcctccgcactcgacttgctagggctgtcttttggagtctgcggctccggatgcgacttggtagagcctccaggccgttggctcaagctggggtgggtggagacgtttcctgcagaaggccgtactccagcttcttcttgcttgacgctttcggtggccaagagcggcacggctcccgccgctgcgacgttcaggaggaccaaggcaaccacgaaccgcatcctgctcggatagcgcttccgccctct

SEQ ID NO: 11107 - RNA, 4834 nt, Homo sapiens
  source 1..4834: mol_type = other RNA
ctgaatagctgggactacaggtgcacgtcaccatgcccggctaatttttgtatttttattagagacggggtttcaccatgttggccaggatggtctcgatctcttgacctcgtgatccccccgcctcggcctcccaaagcgctgggattacagggggagccaccgcgcccggcctttcttcagtgcaatttctaaagagaaacttaaatcctgttgtattctttcaacacaagcaatgatacttctcagagtctgctcaaaagctcagctctgtggactccgtgacaaaatgtacgcgtccactgccgaccctcttggtttctgaaaccaacctttcttcctgctctcctctttaagagcaaaccccaacatgtataaggtcacagcaagtggtagccaggaaaagctgtgggacccctcatttgagtcacatccatatggcatggagaaagaaaacctctctgccagaaggaactgaactctggaagtcctaaggaaggtcaccatgatcagcagataggaaagcattgccaagggctgtccctcaagagcttagttttcttagggagaccagaaagacatcagatcctgactgccctgttttgctcaagttctgaaatgagtggcatgatgaagagctggtggagctgagggaaagagtcaaccatgtggggtggggtagtgaggaaggtgtatgaggaaacaaactgggccctgacgaaacaggcggattggggaaggagaaagaaggaagggagagaaacctaaccaaagaaacatgggaagctggaaagtcgagggcacagccggaataaaggcacagatgggcaccccacaggaggggccttggccaggttgggatgcagagaaaaacaggcaggagggtgtcaatctatagcatcctgaaccccaaaaggtctgtaactggattctctaagccttgagaagttcacaccaaagcttcagaccagggaaaatattttggaaagatcagtctttccaagagtgagctcctttccaagaagctggacaggaaacccaataaatgtggatctgaaaaaacaaaatccaagagagaagcaaaatgggctgggggtgtgcaataagagaagcaaggaaaatggaaagactgtagctgaggatcttttattaaaaaaaaatggatgggactttggtgatgagagagaaaaagggcaaaagtctgcagttaggaatttaggtgaccgaagactgtcctagacagttgggagggacaggctgatggacagaagagagaaattcctttcaatgacaaccaagctgaactattcgataccagcagaactgggttctttagggattaagccaagacaaagacttgggaatcactcactccgaggatgaagaatgggttaatggctgaggagacagtcaaaggaatagagaggcctggctttgagggcctcttcaccaccagcacaagataaggcaaaggaccatttgtcagagacaccaagaaaggggaatttccatttggatggtcaatagtgtccagttctgccaaggacaagactaagctttgagaaaaagccatggatttggtgattggataactggtaacctttagaaaagtttagttgacagacagagaccgaagtgagttagtaaaagtcatgaagagaatgaatggcaacttaagggaagcaacatactggagaagttgagcagcgggatgaataacaaataggacagatgggaacagaaaaatctgggtgcatacgaaggtggatggaaaggagctggtacagatgggcacaaccagaaaacatgaggaggggaaaggaagggaaaaggaaggcaggcagggagagagacgtgaaatagccacagtcttaggggatgctagagaagcctagaagattcctcaggttggtgcaaagtattataagactaacgcatcagtacagagaatgacccaagaagggtaggagttcattccttaccttcataaagtaggctatccgccaagaatgaaaatgtcaactcaaagctatgggctgttttaagcaaggtggaagataatataagaagcatggtcctttcttcagacttactgccttgacagcacagaattcatcttatttccctcatctcccaagttatttgtatttccctgagatcagctcagaaacaactctctttaggctctctacaatgcggtagagcatgattagaaaagataaaccttcaaacaatagtgttgtccaagacactaccctcacttatcccaggggaacccacggaatttcttcatttgtattaactcctgacatggcatggaagaagaatttttatcaaatacccttggcatcttatatcagattaaaggaccattaaatacactgaggtaaaattggcagagagtatagtttctattaataaatctaagtctattttgtctgttttaggcaacaaaggcaaaatggactttgtgggaaatgtatctcataaaagccctttggaaaaactgcagaccaaaaccaaaaccctccttcatgttttctcgcatgaaacataaacttgccctatttcaaaaagttcctactgagtatgattgtgtgaaagatcacactacttcaaatcatatttattttaaaaatctgtgatgggacagtggcctcactgccaggaagcccaagttctgttttatgctcggtacaactaagtggaagttgattcactttgtctcaagctacataaaataatcagaaaatcaagaagatctcatgctagacaggttagacttgcacccaaaaaagcatctttttttttaacctgctgttttggtttgctgctgaagtctttgaagagaattatgtattcaaagtagctctttgcccattggcatttccccatcttctatgtcttctgtagggcacatcccccccaaagtaagaggccttagtagaaaagcacttccacctgcagttttcccctaggtctgcagagagaaacagtgcagagtgcaatgccacagtcaaggaccaactttcctacagagcccgggccccagggagggtggtcagcagcgcagcctgcccaggctgggatctccctttggtcatagccgtgtttccatatacccctccactcaccctcagaggaggaacggatggaagccaccagcataaataaagggaacacagaagaacaatgtcaccaaagtgcaggtgcaaagcccaaagcagccccctacctctgccagcccagacccgccactaaattctagaggagggtgtctctcaggtcacagtacttttttcttcatttcttttgatttagaaacaaatcagcagggaggacaaggttctcaaggacaaaaaaatcaaagctgaaacgagagcagcacaatccattggtgacgttcatctttttccagaggaatataccattctgttaggacttaggggaaaaaagatcttttaggaggtgcagggaaaacattcagaattaagacatacttctggtccaaacgttggtagtcactggcctttggccgccgggtgactttagatctttttccttccaggacaaaagcaatgatcttccgcttgttgtgatgagcgatatagaggacagccacaagaatggctgcagtcaccagatatgcaaagaagtggctgctctccgcgctgccatttccagaaccgttcggataaaggtcatccttctcgctacccgtggaatccgaaagtgtcccttcacggttctcactggaggcagaaccggacatcttttctttctcttctttgggcggtgagccctcctcgggtcctgtatcatcatcttcagcctctttgggctccacatcctcagtaggctctgaagacttaacttcctcctgcgggggagaaatgaggtcagtttcctccccagattcggttttgaaagcatgaggagaaagcttccctttgtcagcaagctggtttgtgtcagccttggggagctccttgttatcagaagggttggagatgggcttggaatggtctttccgggaaggctgctctggaaccaccttgttagggctgtcttttgaggtctgctcctccgcacccgacttgctgggcccgtctattgggccctgctcctctgcaccggacttgttagagccgtcttttggagtctgcttctccgcacccgacttgttagggacgtcttttggggtctgatcctccgcacccgacttgctggagccgtcttttggggtctggccgtccgcacccgacttattagggacatcttttgtggtctgcgcctccgaacctgacttgctagggctgtctttttgggtctttgcctccgcacccgacctgttggggctgtcttctggggtctgcgcctccgcacccgatttgccagtgctgtcttttggagtctgcagctccggatgcgacttactagtgctgtcttttgtggtctgcgcctccgaacccgacttgctagtgctgcctttttgggtctttgcctccgcacccgacttgttggagctgtctttttgggtctttgcctccgcacccgacttgttgggggtgtcttctggggtctgcgcctccgcactcgacttgctagggctgtcttttggagtctgcggctccggatgcgacttggtagagcctccaggccgttggctcaagctggggtgggtggagacgtttcctgcagaaggccgtactccagcttcttcttgcttgacgctttcggtggccaagagcggcacggctcccgccgctgcgacgttcaggaggaccaaggcaaccacgaaccgcatcctgctcggatagcgcttccgccctct

SEQ ID NO: 11108 - RNA, 4776 nt, Homo sapiens
  source 1..4776: mol_type = other RNA
ctgaatagctgggactacaggtgcacgtcaccatgcccggctaatttttgtatttttattagagacggggtttcaccatgttggccaggatggtctcgatctcttgacctcgtgatccccccgcctcggcctcccaaagcgctgggattacagggggagccaccgcgcccggcctttcttcagtgcaatttctaaagagaaacttaaatcctgttgtattctttcaacacaagcaatgatacttctcagagtctgctcaaaagctcagctctgtggactccgtgacaaaatgtacgcgtccactgccgaccctcttggtttctgaaaccaacctttcttcctgctctcctctttaagagcaaaccccaacatgtataaggtcacagcaagtggtagccaggaaaagctgtgggacccctcatttgagtcacatccatatggcatggagaaagaaaacctctctgccagaaggaactgaactctggaagtcctaaggaaggtcaccatgatcagcagataggaaagcattgccaagggctgtccctcaagagcttagttttcttagggagaccagaaagacatcagatcctgactgccctgttttgctcaagttctgaaatgagtggcatgatgaagagctggtggagctgagggaaagagtcaaccatgtggggtggggtagtgaggaaggtgtatgaggaaacaaactgggccctgacgaaacaggcggattggggaaggagaaagaaggaagggagagaaacctaaccaaagaaacatgggaagctggaaagtcgagggcacagccggaataaaggcacagatgggcaccccacaggaggggccttggccaggttgggatgcagagaaaaacaggcaggagggtgtcaatctatagcatcctgaaccccaaaaggtctgtaactggattctctaagccttgagaagttcacaccaaagcttcagaccagggaaaatattttggaaagatcagtctttccaagagtgagctcctttccaagaagctggacaggaaacccaataaatgtggatctgaaaaaacaaaatccaagagagaagcaaaatgggctgggggtgtgcaataagagaagcaaggaaaatggaaagactgtagctgaggatcttttattaaaaaaaaatggatgggactttggtgatgagagagaaaaagggcaaaagtctgcagttaggaatttaggtgaccgaagactgtcctagacagttgggagggacaggctgatggacagaagagagaaattcctttcaatgacaaccaagctgaactattcgataccagcagaactgggttctttagggattaagccaagacaaagacttgggaatcactcactccgaggatgaagaatgggttaatggctgaggagacagtcaaaggaatagagaggcctggctttgagggcctcttcaccaccagcacaagataaggcaaaggaccatttgtcagagacaccaagaaaggggaatttccatttggatggtcaatagtgtccagttctgccaaggacaagactaagctttgagaaaaagccatggatttggtgattggataactggtaacctttagaaaagtttagttgacagacagagaccgaagtgagttagtaaaagtcatgaagagaatgaatggcaacttaagggaagcaacatactggagaagttgagcagcgggatgaataacaaataggacagatgggaacagaaaaatctgggtgcatacgaaggtggatggaaaggagctggtacagatgggcacaaccagaaaacatgaggaggggaaaggaagggaaaaggaaggcaggcagggagagagacgtgaaatagccacagtcttaggggatgctagagaagcctagaagattcctcaggttggtgcaaagtattataagactaacgcatcagtacagagaatgacccaagaagggtaggagttcattccttaccttcataaagtaggctatccgccaagaatgaaaatgtcaactcaaagctatgggctgttttaagcaaggtggaagataatataagaagcatggtcctttcttcagacttactgccttgacagcacagaattcatcttatttccctcatctcccaagttatttgtatttccctgagatcagctcagaaacaactctctttaggctctctacaatgcggtagagcatgattagaaaagataaaccttcaaacaatagtgttgtccaagacactaccctcacttatcccaggggaacccacggaatttcttcatttgtattaactcctgacatggcatggaagaagaatttttatcaaatacccttggcatcttatatcagattaaaggaccattaaatacactgaggtaaaattggcagagagtatagtttctattaataaatctaagtctattttgtctgttttaggcaacaaaggcaaaatggactttgtgggaaatgtatctcataaaagccctttggaaaaactgcagaccaaaaccaaaaccctccttcatgttttctcgcatgaaacataaacttgccctatttcaaaaagttcctactgagtatgattgtgtgaaagatcacactacttcaaatcatatttattttaaaaatctgtgatgggacagtggcctcactgccaggaagcccaagttctgttttatgctcggtacaactaagtggaagttgattcactttgtctcaagctacataaaataatcagaaaatcaagaagatctcatgctagacaggttagacttgcacccaaaaaagcatctttttttttaacctgctgttttggtttgctgctgaagtctttgaagagaattatgtattcaaagtagctctttgcccattggcatttccccatcttctatgtcttctgtagggcacatcccccccaaagtaagaggccttagtagaaaagcacttccacctgcagttttcccctaggtctgcagagagaaacagtgcagagtgcaatgccacagtcaaggaccaactttcctacagagcccgggccccagggagggtggtcagcagcgcagcctgcccaggctgggatctccctttggtcatagccgtgtttccatatacccctccactcaccctcagaggaggaacggatggaagccaccagcataaataaagggaacacagaagaacaatgtcaccaaagtgcaggtgcaaagcccaaagcagccccctacctctgccagcccagacccgccactaaattctagaggagggtgtctctcaggtcacagtacttttttcttcatttcttttgatttagaaacaaatcagcagggaggacaaggttctcaaggacaaaaaaatcaaagctgaaacgagagcagcacaatccattggtgacgttcatctttttccagaggaatataccattctgttaggacttctggtccaaacgttggtagtcactggcctttggccgccgggtgactttagatctttttccttccaggacaaaagcaatgatcttccgcttgttgtgatgagcgatatagaggacagccacaagaatggctgcagtcaccagatatgcaaagaagtggctgctctccgcgctgccatttccagaaccgttcggataaaggtcatccttctcgctacccgtggaatccgaaagtgtcccttcacggttctcactggaggcagaaccggacatcttttctttctcttctttgggcggtgagccctcctcgggtcctgtatcatcatcttcagcctctttgggctccacatcctcagtaggctctgaagacttaacttcctcctgcgggggagaaatgaggtcagtttcctccccagattcggttttgaaagcatgaggagaaagcttccctttgtcagcaagctggtttgtgtcagccttggggagctccttgttatcagaagggttggagatgggcttggaatggtctttccgggaaggctgctctggaaccaccttgttagggctgtcttttgaggtctgctcctccgcacccgacttgctgggcccgtctattgggccctgctcctctgcaccggacttgttagagccgtcttttggagtctgcttctccgcacccgacttgttagggacgtcttttggggtctgatcctccgcacccgacttgctggagccgtcttttggggtctggccgtccgcacccgacttattagggacatcttttgtggtctgcgcctccgaacctgacttgctagggctgtctttttgggtctttgcctccgcacccgacctgttggggctgtcttctggggtctgcgcctccgcacccgatttgccagtgctgtcttttggagtctgcagctccggatgcgacttactagtgctgtcttttgtggtctgcgcctccgaacccgacttgctagtgctgcctttttgggtctttgcctccgcacccgacttgttggagctgtctttttgggtctttgcctccgcacccgacttgttgggggtgtcttctggggtctgcgcctccgcactcgacttgctagggctgtcttttggagtctgcggctccggatgcgacttggtagagcctccaggccgttggctcaagctggggtgggtggagacgtttcctgcagaaggccgtactccagcttcttcttgcttgacgctttcggtggccaagagcggcacggctcccgccgctgcgacgttcaggaggaccaaggcaaccacgaaccgcatcctgctcggatagcgcttccgccctct

SEQ ID NO: 11109 - RNA, 4602 nt, Homo sapiens
  source 1..4602: mol_type = other RNA
ctgaatagctgggactacaggtgcacgtcaccatgcccggctaatttttgtatttttattagagacggggtttcaccatgttggccaggatggtctcgatctcttgacctcgtgatccccccgcctcggcctcccaaagcgctgggattacagggggagccaccgcgcccggcctttcttcagtgcaatttctaaagagaaacttaaatcctgttgtattctttcaacacaagcaatgatacttctcagagtctgctcaaaagctcagctctgtggactccgtgacaaaatgtacgcgtccactgccgaccctcttggtttctgaaaccaacctttcttcctgctctcctctttaagagcaaaccccaacatgtataaggtcacagcaagtggtagccaggaaaagctgtgggacccctcatttgagtcacatccatatggcatggagaaagaaaacctctctgccagaaggaactgaactctggaagtcctaaggaaggtcaccatgatcagcagataggaaagcattgccaagggctgtccctcaagagcttagttttcttagggagaccagaaagacatcagatcctgactgccctgttttgctcaagttctgaaatgagtggcatgatgaagagctggtggagctgagggaaagagtcaaccatgtggggtggggtagtgaggaaggtgtatgaggaaacaaactgggccctgacgaaacaggcggattggggaaggagaaagaaggaagggagagaaacctaaccaaagaaacatgggaagctggaaagtcgagggcacagccggaataaaggcacagatgggcaccccacaggaggggccttggccaggttgggatgcagagaaaaacaggcaggagggtgtcaatctatagcatcctgaaccccaaaaggtctgtaactggattctctaagccttgagaagttcacaccaaagcttcagaccagggaaaatattttggaaagatcagtctttccaagagtgagctcctttccaagaagctggacaggaaacccaataaatgtggatctgaaaaaacaaaatccaagagagaagcaaaatgggctgggggtgtgcaataagagaagcaaggaaaatggaaagactgtagctgaggatcttttattaaaaaaaaatggatgggactttggtgatgagagagaaaaagggcaaaagtctgcagttaggaatttaggtgaccgaagactgtcctagacagttgggagggacaggctgatggacagaagagagaaattcctttcaatgacaaccaagctgaactattcgataccagcagaactgggttctttagggattaagccaagacaaagacttgggaatcactcactccgaggatgaagaatgggttaatggctgaggagacagtcaaaggaatagagaggcctggctttgagggcctcttcaccaccagcacaagataaggcaaaggaccatttgtcagagacaccaagaaaggggaatttccatttggatggtcaatagtgtccagttctgccaaggacaagactaagctttgagaaaaagccatggatttggtgattggataactggtaacctttagaaaagtttagttgacagacagagaccgaagtgagttagtaaaagtcatgaagagaatgaatggcaacttaagggaagcaacatactggagaagttgagcagcgggatgaataacaaataggacagatgggaacagaaaaatctgggtgcatacgaaggtggatggaaaggagctggtacagatgggcacaaccagaaaacatgaggaggggaaaggaagggaaaaggaaggcaggcagggagagagacgtgaaatagccacagtcttaggggatgctagagaagcctagaagattcctcaggttggtgcaaagtattataagactaacgcatcagtacagagaatgacccaagaagggtaggagttcattccttaccttcataaagtaggctatccgccaagaatgaaaatgtcaactcaaagctatgggctgttttaagcaaggtggaagataatataagaagcatggtcctttcttcagacttactgccttgacagcacagaattcatcttatttccctcatctcccaagttatttgtatttccctgagatcagctcagaaacaactctctttaggctctctacaatgcggtagagcatgattagaaaagataaaccttcaaacaatagtgttgtccaagacactaccctcacttatcccaggggaacccacggaatttcttcatttgtattaactcctgacatggcatggaagaagaatttttatcaaatacccttggcatcttatatcagattaaaggaccattaaatacactgaggtaaaattggcagagagtatagtttctattaataaatctaagtctattttgtctgttttaggcaacaaaggcaaaatggactttgtgggaaatgtatctcataaaagccctttggaaaaactgcagaccaaaaccaaaaccctccttcatgttttctcgcatgaaacataaacttgccctatttcaaaaagttcctactgagtatgattgtgtgaaagatcacactacttcaaatcatatttattttaaaaatctgtgatgggacagtggcctcactgccaggaagcccaagttctgttttatgctcggtacaactaagtggaagttgattcactttgtctcaagctacataaaataatcagaaaatcaagaagatctcatgctagacaggttagacttgcacccaaaaaagcatctttttttttaacctgctgttttggtttgctgctgaagtctttgaagagaattatgtattcaaagtagctctttgcccattggcatttccccatcttctatgtcttctgtagggcacatcccccccaaagtaagaggccttagtagaaaagcacttccacctgcagttttcccctaggtctgcagagagaaacagtgcagagtgcaatgccacagtcaaggaccaactttcctacagagcccgggccccagggagggtggtcagcagcgcagcctgcccaggctgggatctccctttggtcatagccgtgtttccatatacccctccactcaccctcagaggaggaacggatggaagccaccagcataaataaagggaacacagaagaacaatgtcaccaaagtgcaggtgcaaagcccaaagcagccccctacctctgccagcccagacccgccactaaattctagaggagggtgtctctcaggtcacagtacttttttcttcatttcttttgatttagaaacaaatcagcagggaggacaaggttctcaaggacaaaaaaatcaaagctgaaacgagagcagcacaatccattggtgacgttcatctttttccagaggaatataccattctgttaggacttctggtccaaacgttggtagtcactggcctttggccgccgggtgactttagatctttttccttccaggacaaaagcaatgatcttccgcttgttgtgatgagcgatatagaggacagccacaagaatggctgcagtcaccagatatgcaaagaagtggctgctctccgcgctgccatttccagaaccgttcggataaaggtcatccttctcgctacccgtggaatccgaaagtgtcccttcacggttctcactggaggcagaaccggacatcttttctttctcttctttgggcggtgagccctcctcgggtcctgtatcatcatcttcagcctctttgggctccacatcctcagtaggctctgaagacttaacttcctccttgttagggctgtcttttgaggtctgctcctccgcacccgacttgctgggcccgtctattgggccctgctcctctgcaccggacttgttagagccgtcttttggagtctgcttctccgcacccgacttgttagggacgtcttttggggtctgatcctccgcacccgacttgctggagccgtcttttggggtctggccgtccgcacccgacttattagggacatcttttgtggtctgcgcctccgaacctgacttgctagggctgtctttttgggtctttgcctccgcacccgacctgttggggctgtcttctggggtctgcgcctccgcacccgatttgccagtgctgtcttttggagtctgcagctccggatgcgacttactagtgctgtcttttgtggtctgcgcctccgaacccgacttgctagtgctgcctttttgggtctttgcctccgcacccgacttgttggagctgtctttttgggtctttgcctccgcacccgacttgttgggggtgtcttctggggtctgcgcctccgcactcgacttgctagggctgtcttttggagtctgcggctccggatgcgacttggtagagcctccaggccgttggctcaagctggggtgggtggagacgtttcctgcagaaggccgtactccagcttcttcttgcttgacgctttcggtggccaagagcggcacggctcccgccgctgcgacgttcaggaggaccaaggcaaccacgaaccgcatcctgctcggatagcgcttccgccctct

SEQ ID NO: 11110 - RNA, 4793 nt, Homo sapiens
  source 1..4793: mol_type = other RNA
ctgaatagctgggactacaggtgcacgtcaccatgcccggctaatttttgtatttttattagagacggggtttcaccatgttggccaggatggtctcgatctcttgacctcgtgatccccccgcctcggcctcccaaagcgctgggattacagggggagccaccgcgcccggcctttcttcagtgcaatttctaaagagaaacttaaatcctgttgtattctttcaacacaagcaatgatacttctcagagtctgctcaaaagctcagctctgtggactccgtgacaaaatgtacgcgtccactgccgaccctcttggtttctgaaaccaacctttcttcctgctctcctctttaagagcaaaccccaacatgtataaggtcacagcaagtggtagccaggaaaagctgtgggacccctcatttgagtcacatccatatggcatggagaaagaaaacctctctgccagaaggaactgaactctggaagtcctaaggaaggtcaccatgatcagcagataggaaagcattgccaagggctgtccctcaagagcttagttttcttagggagaccagaaagacatcagatcctgactgccctgttttgctcaagttctgaaatgagtggcatgatgaagagctggtggagctgagggaaagagtcaaccatgtggggtggggtagtgaggaaggtgtatgaggaaacaaactgggccctgacgaaacaggcggattggggaaggagaaagaaggaagggagagaaacctaaccaaagaaacatgggaagctggaaagtcgagggcacagccggaataaaggcacagatgggcaccccacaggaggggccttggccaggttgggatgcagagaaaaacaggcaggagggtgtcaatctatagcatcctgaaccccaaaaggtctgtaactggattctctaagccttgagaagttcacaccaaagcttcagaccagggaaaatattttggaaagatcagtctttccaagagtgagctcctttccaagaagctggacaggaaacccaataaatgtggatctgaaaaaacaaaatccaagagagaagcaaaatgggctgggggtgtgcaataagagaagcaaggaaaatggaaagactgtagctgaggatcttttattaaaaaaaaatggatgggactttggtgatgagagagaaaaagggcaaaagtctgcagttaggaatttaggtgaccgaagactgtcctagacagttgggagggacaggctgatggacagaagagagaaattcctttcaatgacaaccaagctgaactattcgataccagcagaactgggttctttagggattaagccaagacaaagacttgggaatcactcactccgaggatgaagaatgggttaatggctgaggagacagtcaaaggaatagagaggcctggctttgagggcctcttcaccaccagcacaagataaggcaaaggaccatttgtcagagacaccaagaaaggggaatttccatttggatggtcaatagtgtccagttctgccaaggacaagactaagctttgagaaaaagccatggatttggtgattggataactggtaacctttagaaaagtttagttgacagacagagaccgaagtgagttagtaaaagtcatgaagagaatgaatggcaacttaagggaagcaacatactggagaagttgagcagcgggatgaataacaaataggacagatgggaacagaaaaatctgggtgcatacgaaggtggatggaaaggagctggtacagatgggcacaaccagaaaacatgaggaggggaaaggaagggaaaaggaaggcaggcagggagagagacgtgaaatagccacagtcttaggggatgctagagaagcctagaagattcctcaggttggtgcaaagtattataagactaacgcatcagtacagagaatgacccaagaagggtaggagttcattccttaccttcataaagtaggctatccgccaagaatgaaaatgtcaactcaaagctatgggctgttttaagcaaggtggaagataatataagaagcatggtcctttcttcagacttactgccttgacagcacagaattcatcttatttccctcatctcccaagttatttgtatttccctgagatcagctcagaaacaactctctttaggctctctacaatgcggtagagcatgattagaaaagataaaccttcaaacaatagtgttgtccaagacactaccctcacttatcccaggggaacccacggaatttcttcatttgtattaactcctgacatggcatggaagaagaatttttatcaaatacccttggcatcttatatcagattaaaggaccattaaatacactgaggtaaaattggcagagagtatagtttctattaataaatctaagtctattttgtctgttttaggcaacaaaggcaaaatggactttgtgggaaatgtatctcataaaagccctttggaaaaactgcagaccaaaaccaaaaccctccttcatgttttctcgcatgaaacataaacttgccctatttcaaaaagttcctactgagtatgattgtgtgaaagatcacactacttcaaatcatatttattttaaaaatctgtgatgggacagtggcctcactgccaggaagcccaagttctgttttatgctcggtacaactaagtggaagttgattcactttgtctcaagctacataaaataatcagaaaatcaagaagatctcatgctagacaggttagacttgcacccaaaaaagcatctttttttttaacctgctgttttggtttgctgctgaagtctttgaagagaattatgtattcaaagtagctctttgcccattggcatttccccatcttctatgtcttctgtagggcacatcccccccaaagtaagaggccttagtagaaaagcacttccacctgcagttttcccctaggtctgcagagagaaacagtgcagagtgcaatgccacagtcaaggaccaactttcctacagagcccgggccccagggagggtggtcagcagcgcagcctgcccaggctgggatctccctttggtcatagccgtgtttccatatacccctccactcaccctcagaggaggaacggatggaagccaccagcataaataaagggaacacagaagaacaatgtcaccaaagtgcaggtgcaaagcccaaagcagccccctacctctgccagcccagacccgccactaaattctagaggagggtgtctctcaggtcacagtacttttttcttcatttcttttgatttagaaacaaatcagcagggaggacaaggttctcaaggacaaaaaaatcaaagctgaaacgagagcagcacaatccattggtgacgttcatctttttccagaggaatataccattctgttaggacttgggggaaaaaagatcttctggtccaaacgttggtagtcactggcctttggccgccgggtgactttagatctttttccttccaggacaaaagcaatgatcttccgcttgttgtgatgagcgatatagaggacagccacaagaatggctgcagtcaccagatatgcaaagaagtggctgctctccgcgctgccatttccagaaccgttcggataaaggtcatccttctcgctacccgtggaatccgaaagtgtcccttcacggttctcactggaggcagaaccggacatcttttctttctcttctttgggcggtgagccctcctcgggtcctgtatcatcatcttcagcctctttgggctccacatcctcagtaggctctgaagacttaacttcctcctgcgggggagaaatgaggtcagtttcctccccagattcggttttgaaagcatgaggagaaagcttccctttgtcagcaagctggtttgtgtcagccttggggagctccttgttatcagaagggttggagatgggcttggaatggtctttccgggaaggctgctctggaaccaccttgttagggctgtcttttgaggtctgctcctccgcacccgacttgctgggcccgtctattgggccctgctcctctgcaccggacttgttagagccgtcttttggagtctgcttctccgcacccgacttgttagggacgtcttttggggtctgatcctccgcacccgacttgctggagccgtcttttggggtctggccgtccgcacccgacttattagggacatcttttgtggtctgcgcctccgaacctgacttgctagggctgtctttttgggtctttgcctccgcacccgacctgttggggctgtcttctggggtctgcgcctccgcacccgatttgccagtgctgtcttttggagtctgcagctccggatgcgacttactagtgctgtcttttgtggtctgcgcctccgaacccgacttgctagtgctgcctttttgggtctttgcctccgcacccgacttgttggagctgtctttttgggtctttgcctccgcacccgacttgttgggggtgtcttctggggtctgcgcctccgcactcgacttgctagggctgtcttttggagtctgcggctccggatgcgacttggtagagcctccaggccgttggctcaagctggggtgggtggagacgtttcctgcagaaggccgtactccagcttcttcttgcttgacgctttcggtggccaagagcggcacggctcccgccgctgcgacgttcaggaggaccaaggcaaccacgaaccgcatcctgctcggatagcgcttccgccctct

SEQ ID NO: 11111 - RNA, 4834 nt, Homo sapiens
  source 1..4834: mol_type = other RNA
ctgaatagctgggactacaggtgcacgtcaccatgcccggctaatttttgtatttttattagagacggggtttcaccatgttggccaggatggtctcgatctcttgacctcgtgatccccccgcctcggcctcccaaagcgctgggattacagggggagccaccgcgcccggcctttcttcagtgcaatttctaaagagaaacttaaatcctgttgtattctttcaacacaagcaatgatacttctcagagtctgctcaaaagctcagctctgtggactccgtgacaaaatgtacgcgtccactgccgaccctcttggtttctgaaaccaacctttcttcctgctctcctctttaagagcaaaccccaacatgtataaggtcacagcaagtggtagccaggaaaagctgtgggacccctcatttgagtcacatccatatggcatggagaaagaaaacctctctgccagaaggaactgaactctggaagtcctaaggaaggtcaccatgatcagcagataggaaagcattgccaagggctgtccctcaagagcttagttttcttagggagaccagaaagacatcagatcctgactgccctgttttgctcaagttctgaaatgagtggcatgatgaagagctggtggagctgagggaaagagtcaaccatgtggggtggggtagtgaggaaggtgtatgaggaaacaaactgggccctgacgaaacaggcggattggggaaggagaaagaaggaagggagagaaacctaaccaaagaaacatgggaagctggaaagtcgagggcacagccggaataaaggcacagatgggcaccccacaggaggggccttggccaggttgggatgcagagaaaaacaggcaggagggtgtcaatctatagcatcctgaaccccaaaaggtctgtaactggattctctaagccttgagaagttcacaccaaagcttcagaccagggaaaatattttggaaagatcagtctttccaagagtgagctcctttccaagaagctggacaggaaacccaataaatgtggatctgaaaaaacaaaatccaagagagaagcaaaatgggctgggggtgtgcaataagagaagcaaggaaaatggaaagactgtagctgaggatcttttattaaaaaaaaatggatgggactttggtgatgagagagaaaaagggcaaaagtctgcagttaggaatttaggtgaccgaagactgtcctagacagttgggagggacaggctgatggacagaagagagaaattcctttcaatgacaaccaagctgaactattcgataccagcagaactgggttctttagggattaagccaagacaaagacttgggaatcactcactccgaggatgaagaatgggttaatggctgaggagacagtcaaaggaatagagaggcctggctttgagggcctcttcaccaccagcacaagataaggcaaaggaccatttgtcagagacaccaagaaaggggaatttccatttggatggtcaatagtgtccagttctgccaaggacaagactaagctttgagaaaaagccatggatttggtgattggataactggtaacctttagaaaagtttagttgacagacagagaccgaagtgagttagtaaaagtcatgaagagaatgaatggcaacttaagggaagcaacatactggagaagttgagcagcgggatgaataacaaataggacagatgggaacagaaaaatctgggtgcatacgaaggtggatggaaaggagctggtacagatgggcacaaccagaaaacatgaggaggggaaaggaagggaaaaggaaggcaggcagggagagagacgtgaaatagccacagtcttaggggatgctagagaagcctagaagattcctcaggttggtgcaaagtattataagactaacgcatcagtacagagaatgacccaagaagggtaggagttcattccttaccttcataaagtaggctatccgccaagaatgaaaatgtcaactcaaagctatgggctgttttaagcaaggtggaagataatataagaagcatggtcctttcttcagacttactgccttgacagcacagaattcatcttatttccctcatctcccaagttatttgtatttccctgagatcagctcagaaacaactctctttaggctctctacaatgcggtagagcatgattagaaaagataaaccttcaaacaatagtgttgtccaagacactaccctcacttatcccaggggaacccacggaatttcttcatttgtattaactcctgacatggcatggaagaagaatttttatcaaatacccttggcatcttatatcagattaaaggaccattaaatacactgaggtaaaattggcagagagtatagtttctattaataaatctaagtctattttgtctgttttaggcaacaaaggcaaaatggactttgtgggaaatgtatctcataaaagccctttggaaaaactgcagaccaaaaccaaaaccctccttcatgttttctcgcatgaaacataaacttgccctatttcaaaaagttcctactgagtatgattgtgtgaaagatcacactacttcaaatcatatttattttaaaaatctgtgatgggacagtggcctcactgccaggaagcccaagttctgttttatgctcggtacaactaagtggaagttgattcactttgtctcaagctacataaaataatcagaaaatcaagaagatctcatgctagacaggttagacttgcacccaaaaaagcatctttttttttaacctgctgttttggtttgctgctgaagtctttgaagagaattatgtattcaaagtagctctttgcccattggcatttccccatcttctatgtcttctgtagggcacatcccccccaaagtaagaggccttagtagaaaagcacttccacctgcagttttcccctaggtctgcagagagaaacagtgcagagtgcaatgccacagtcaaggaccaactttcctacagagcccgggccccagggagggtggtcagcagcgcagcctgcccaggctgggatctccctttggtcatagccgtgtttccatatacccctccactcaccctcagaggaggaacggatggaagccaccagcataaataaagggaacacagaagaacaatgtcaccaaagtgcaggtgcaaagcccaaagcagccccctacctctgccagcccagacccgccactaaattctagaggagggtgtctctcaggtcacagtacttttttcttcatttcttttgatttagaaacaaatcagcagggaggacaaggttctcaaggacaaaaaaatcaaagctgaaacgagagcagcacaatccattggtgacgttcatctttttccagaggaatataccattctgttaggacttgggggaaaaaagatcttttaggaggtgcagggaaaacattcagaattaagacatacttctggtccaaacgttggtagtcactggcctttggccgccgggtgactttagatctttttccttccaggacaaaagcaatgatcttccgcttgttgtgatgagcgatatagaggacagccacaagaatggctgcagtcaccagatatgcaaagaagtggctgctctccgcgctgccatttccagaaccgttcggataaaggtcatccttctcgctacccgtggaatccgaaagtgtcccttcacggttctcactggaggcagaaccggacatcttttctttctcttctttgggcggtgagccctcctcgggtcctgtatcatcatcttcagcctctttgggctccacatcctcagtaggctctgaagacttaacttcctcctgcgggggagaaatgaggtcagtttcctccccagattcggttttgaaagcatgaggagaaagcttccctttgtcagcaagctggtttgtgtcagccttggggagctccttgttatcagaagggttggagatgggcttggaatggtctttccgggaaggctgctctggaaccaccttgttagggctgtcttttgaggtctgctcctccgcacccgacttgctgggcccgtctattgggccctgctcctctgcaccggacttgttagagccgtcttttggagtctgcttctccgcacccgacttgttagggacgtcttttggggtctgatcctccgcacccgacttgctggagccgtcttttggggtctggccgtccgcacccgacttattagggacatcttttgtggtctgcgcctccgaacctgacttgctagggctgtctttttgggtctttgcctccgcacccgacctgttggggctgtcttctggggtctgcgcctccgcacccgatttgccagtgctgtcttttggagtctgcagctccggatgcgacttactagtgctgtcttttgtggtctgcgcctccgaacccgacttgctagtgctgcctttttgggtctttgcctccgcacccgacttgttggagctgtctttttgggtctttgcctccgcacccgacttgttgggggtgtcttctggggtctgcgcctccgcactcgacttgctagggctgtcttttggagtctgcggctccggatgcgacttggtagagcctccaggccgttggctcaagctggggtgggtggagacgtttcctgcagaaggccgtactccagcttcttcttgcttgacgctttcggtggccaagagcggcacggctcccgccgctgcgacgttcaggaggaccaaggcaaccacgaaccgcatcctgctcggatagcgcttccgccctct

SEQ ID NO: 11112 - RNA, 4848 nt, Homo sapiens
  source 1..4848: mol_type = other RNA
ctgaatagctgggactacaggtgcactaccacacctggctaagttttaaaatttttgtagagatagggtcttgccatgttgccaggttggtctcaaactcctagcctcaagcaatactcctatctcaggctcccaaagtgctgggattataggcatgagccactgtatctggcctctggggaaaacttttagaaatatacttttaatttttgaaagaaaattaaaccaaacaaaaatcaaatccctaaaactgagtattcccatttactaactggctaaaactgatgatgaaagaagaaaaagtaccttccgatagaaataaagcattatagatcagtgctatttataatttattacttatcaaagtaactccagctttcttatagcaattcaataagccctctcctagaactcaggggcttttaaatttatgtttttactaagaaaacctttttaaaaaaaatccctaagctatatgtttttaaaacatttaaaattgattttttaaattttgaaagtgaaattataaccatcttcaaaacatacagtaaaatgtattacgtagacaagtatcaattatttcaaacagcatgacaatttaactacaaataatttcaaatcctaacaaatataattacctaatgtttaagtaattttataaataaattaccaaattagaagacagtattggttgactacattttacaaactataagaatatatcccacacttcatatattttaacaccctggggtatttttctgcattaataaaattcattctattataaattttcaggaattctttctgatgtaccaagatttcatatgaaaaagcagaagctatttttttatttctgatataaaacagtaagtatgaacccaatgtagaaatctgaagttagacaattccctttggcagaaaacaattataaacaggtcttaatataaatagaatccataagcccataaaaagggaagtacacaaccctgtgtttcttaacaccgaaagaatcatcagtacacagatttaaaatcatttttatctctcgacagcctgcaacacaaaattacatatggcaaaaaataatttttaacttgagaaagaaaaaaacttctgcacatataaactttcaccgatgtgccaatatatactatatatttatatatatatatatgtgtcatgttttattattctaaaactacattatttataatggctgatcccaatttagtgggtgtgcagtaattatattggctcaaagacatgctgaattaaacttttataattgagatcacaattatacatgaaatacacaaacattaaaataagtttattaaatagagtttgggagaaaaaaagtaagaaattccatatatatgcaaatgttgactattatcgagagcagctttggattttttttaaatgttttttaaaaattattattttgtaaataacagaagatttgtttccaaaaagtaaggtgccattcagaagtatataattgaattaacataaaggaaaatactgaataaaaaacagaacatgagatattaaaggttaaaactttctgttcagttatttgtatctgaagttaagacaatgacataaactgagctttcaaatactgctaatttttccacttaaatgtagatcaagtaccatatagactattttgttctagaataaagtttctttgaaaaaggaacatatttataatcaaatttctgtagataaatggcaaaattttcagagaactagcttgaaatggatttagtagaaagaatgactgcttcctttaaaaaaacaaatatagaaatcttgcttccacgtaactttttaaaaactaatgtccattgtttttcccaatctgaatatgtttccatacatgtatgtatttgcaatttctattttccaatatgtaaaaagttggtagacaatgaagtagtgtgcaaatttttaggagagaaaacaatccctactggtttactaccaaactctcacagttatatagaatctattagcactataaactaactcaaaatgcaggcttcagaaaaactgcttcaatagcctccctatcaatctgtcgccttctatgaagtcttcacctgctattattccacaggctgagaattacttctgaaagaaatggtcaattttttcaacagcttggtatgttgacagcttagcaacggtacttgaatcacctctttaaaaaaacaacacaccactaaaaacacacttatcatccatgcttggtatatctcacaacaaattattaggaatgtctcatggttcaaattcacacgcaatcccataaaaaggatatgcagcatctctgcacaccacattgcaggaagaaaaacaaatggaccatatcttcattagagaatagccaaaatcacttgaaaaggttattagtgacaattctaaataccagagatacatgtaggaaagaaaatgtttttcctcagggaatggaaatgttttgtgggacattccttcacagttggcatgactgtttgggggactgactaaatgctttatcacacatctgcatttacaaggtcttcactgttaatcacagaaaacatttttgttccttccagattgctcttgcttctgtagacaattatatgctaattattattcaacataacagtgagagcaaaagtgacaatactgcaaacacaaccgcaatttaaggagccaaaaagaaatatgctggcaagctaaatgcttacacacaaaaaagttagacttttaaagtgtgtgagaaactctgaaaaaaatatttcaagttcttcagtgctcttatgacattttagggggaaacagtggtttctttaaaataatattttaatcctcctatctcatactgtttataagtatgagatacttttgacaaactcactctgtcgatcatgctactgcactccagcctgggtgacagagcgagtttgtcataagtatctcatactgtttgtcataaggctacttaatgagtatctagatttatgtagagaaatctgaaagtaagacaaaactaactgaaagcatctttaagctgcctctgatgaaaagattgacttcaaacaaactggactgaaaaaaaaaaaaaaaaaaaaccttttatggccttgtagaataagagaggtttttgtgctttatttattcatggtccttttgagttgagagggaaaaaagttttaatattttcaggttggtatcacaaggactgaataatacacttatgaaggctttcaagaaaatgcttgatttgtttctaaaggagaggctgctgatggtaatttgtgtgctgctgtgcaactggatgagctggaactgtcaccggaaagcctgccagttgaggcaaattggaagtagtgttctgataagatgacatatccacagacatccccatttgctgtgtgtaagcagttgtaccagtagctgactgtaggttagagttctggttcatataagtaggattggaaacagtgtcttgtccagtgcttaaatatgaagtttgagcaggctgtgctgtcactgaggaattcacatttggaggcagagatctcagtggaccaatttgatcgggtcctaggctatagctttgggcaacagttacttggtgaatgctctgacccatatagtttccaccatgtgattgaactggatatgtctatcaatttcttcaagtttttcatctatcattggacccatctgttggcagatatcttctaaatccaaaaggtcttgggagtctggttttgaatctgttggatctatactctgaagtacctgcagggctctatccatcttatcctcatctatataaacaggctcaggctctgatttcttaatttcctccacatcatcatcaattacattcaatttgtccacagccgctgcctcagtctctatgtttaaattagttgttacaaaattggatgggaaaagtcctattcctctgtgattttctcctttccaccaattggcatcactgtcatccaaaacaataattatttcaccatgtttaaaggtgagttcattgtcctcaacagcttcaaaatcatataaagctctcactttccgtgcaaccttattatttaactgaatttctgaagatggatataaggattttgtttctgtgtgttgctgtttctgttcttgcagcgataattcaatagctttagctatgtcttcatcctctttgtttttgttcgatgacgtaccattcttggcagcagctgagacagtctgagaacctgctggaggaaaagtaattccttcttctttcatagatttaatagttgcagatatcagactaaactgagggtccttctgaaattcttctgaccactccaccattaaagatttcagtttttcacatactttaggatgtgccttatttttaatcacagcacgtacttctgttgcaaaatcacgggaacatacttctaaatgaaatatctttccacagtttgccacacaagccccaagaagagttagtgcttgcagagcaacatgtggaaccttatgatttacccttttcattatggcttttaggcaatctttcgctccattaggagtacttccaactttgtcacatatgtccataataagactccaatcttctgtagtgttgtactcattcgtggctttttccacgtcttgctcgaaggggttggcggtgaacaaaggcatctcgccggcgcccgagccctagtcgctgctgtctagctgacactcagcaactgctacccgccgggtgacccgcggccgcggctccctagaccgctccgcttcggcctccgtccctgcacttccgccaccgcacct

SEQ ID NO: 11113 - RNA, 4988 nt, Homo sapiens
  source 1..4988: mol_type = other RNA
ctgaatagctgggactacaggtgcactaccacacctggctaagttttaaaatttttgtagagatagggtcttgccatgttgccaggttggtctcaaactcctagcctcaagcaatactcctatctcaggctcccaaagtgctgggattataggcatgagccactgtatctggcctctggggaaaacttttagaaatatacttttaatttttgaaagaaaattaaaccaaacaaaaatcaaatccctaaaactgagtattcccatttactaactggctaaaactgatgatgaaagaagaaaaagtaccttccgatagaaataaagcattatagatcagtgctatttataatttattacttatcaaagtaactccagctttcttatagcaattcaataagccctctcctagaactcaggggcttttaaatttatgtttttactaagaaaacctttttaaaaaaaatccctaagctatatgtttttaaaacatttaaaattgattttttaaattttgaaagtgaaattataaccatcttcaaaacatacagtaaaatgtattacgtagacaagtatcaattatttcaaacagcatgacaatttaactacaaataatttcaaatcctaacaaatataattacctaatgtttaagtaattttataaataaattaccaaattagaagacagtattggttgactacattttacaaactataagaatatatcccacacttcatatattttaacaccctggggtatttttctgcattaataaaattcattctattataaattttcaggaattctttctgatgtaccaagatttcatatgaaaaagcagaagctatttttttatttctgatataaaacagtaagtatgaacccaatgtagaaatctgaagttagacaattccctttggcagaaaacaattataaacaggtcttaatataaatagaatccataagcccataaaaagggaagtacacaaccctgtgtttcttaacaccgaaagaatcatcagtacacagatttaaaatcatttttatctctcgacagcctgcaacacaaaattacatatggcaaaaaataatttttaacttgagaaagaaaaaaacttctgcacatataaactttcaccgatgtgccaatatatactatatatttatatatatatatatgtgtcatgttttattattctaaaactacattatttataatggctgatcccaatttagtgggtgtgcagtaattatattggctcaaagacatgctgaattaaacttttataattgagatcacaattatacatgaaatacacaaacattaaaataagtttattaaatagagtttgggagaaaaaaagtaagaaattccatatatatgcaaatgttgactattatcgagagcagctttggattttttttaaatgttttttaaaaattattattttgtaaataacagaagatttgtttccaaaaagtaaggtgccattcagaagtatataattgaattaacataaaggaaaatactgaataaaaaacagaacatgagatattaaaggttaaaactttctgttcagttatttgtatctgaagttaagacaatgacataaactgagctttcaaatactgctaatttttccacttaaatgtagatcaagtaccatatagactattttgttctagaataaagtttctttgaaaaaggaacatatttataatcaaatttctgtagataaatggcaaaattttcagagaactagcttgaaatggatttagtagaaagaatgactgcttcctttaaaaaaacaaatatagaaatcttgcttccacgtaactttttaaaaactaatgtccattgtttttcccaatctgaatatgtttccatacatgtatgtatttgcaatttctattttccaatatgtaaaaagttggtagacaatgaagtagtgtgcaaatttttaggagagaaaacaatccctactggtttactaccaaactctcacagttatatagaatctattagcactataaactaactcaaaatgcaggcttcagaaaaactgcttcaatagcctccctatcaatctgtcgccttctatgaagtcttcacctgctattattccacaggctgagaattacttctgaaagaaatggtcaattttttcaacagcttggtatgttgacagcttagcaacggtacttgaatcacctctttaaaaaaacaacacaccactaaaaacacacttatcatccatgcttggtatatctcacaacaaattattaggaatgtctcatggttcaaattcacacgcaatcccataaaaaggatatgcagcatctctgcacaccacattgcaggaagaaaaacaaatggaccatatcttcattagagaatagccaaaatcacttgaaaaggttattagtgacaattctaaataccagagatacatgtaggaaagaaaatgtttttcctcagggaatggaaatgttttgtgggacattccttcacagttggcatgactgtttgggggactgactaaatgctttatcacacatctgcatttacaaggtcttcactgttaatcacagaaaacatttttgttccttccagattgctcttgcttctgtagacaattatatgctaattattattcaacataacagtgagagcaaaagtgacaatactgcaaacacaaccgcaatttaaggagccaaaaagaaatatgctggcaagctaaatgcttacacacaaaaaagttagacttttaaagtgtgtgagaaactctgaaaaaaatatttcaagttcttcagtgctcttatgacattttagggggaaacagtggtttctttaaaataatattttaatcctcctatctcatactgtttataagtatgagatacttttgacaaactcactctgtcgatcatgctactgcactccagcctgggtgacagagcgagtttgtcataagtatctcatactgtttgtcataaggctacttaatgagtatctagatttatgtagagaaatctgaaagtaagacaaaactaactgaaagcatctttaagctgcctctgatgaaaagattgacttcaaacaaactggactgaaaaaaaaaaaaaaaaaaaaccttttatggccttgtagaataagagaggtttttgtgctttatttattcatggtccttttgagttgagagggaaaaaagttttaatattttcaggttggtatcacaaggactgaataatacacttatgaaggctttcaagaaaatgcttgatttgtttctaaaggagaggctgctgatggtaatttgtgtgctgctgtgcaactggatgagctggaactgtcaccggaaagcctgccagttgaggcaaattggaagtagtgttctgataagatgacatatccacagacatccccatttgctgtgtgtaagcagttgtaccagtagctgactgtaggttagagttctggttcatataagtaggattggaaacagtgtcttgtccagtgcttaaatatgaagtttgagcaggctgtgctgtcactgaggaattcacatttggaggcagagatctcagtggaccaatttgatcgggtcctaggctatagctttgggcaacagttacttggtgaatgctctgacccatatagtttccaccatgtgattgaactggatatgtctgcattggaaccccagatgatgcaggtgggtaatgtgctggagggtggagctttgaatagactgagtacactggtgcttcattcaccaatttgttatatagttccagagcttccaggactttaacattcaattcagacaattctgaatgcttcctatcaatttcttcaagtttttcatctatcattggacccatctgttggcagatatcttctaaatccaaaaggtcttgggagtctggttttgaatctgttggatctatactctgaagtacctgcagggctctatccatcttatcctcatctatataaacaggctcaggctctgatttcttaatttcctccacatcatcatcaattacattcaatttgtccacagccgctgcctcagtctctatgtttaaattagttgttacaaaattggatgggaaaagtcctattcctctgtgattttctcctttccaccaattggcatcactgtcatccaaaacaataattatttcaccatgtttaaaggtgagttcattgtcctcaacagcttcaaaatcatataaagctctcactttccgtgcaaccttattatttaactgaatttctgaagatggatataaggattttgtttctgtgtgttgctgtttctgttcttgcagcgataattcaatagctttagctatgtcttcatcctctttgtttttgttcgatgacgtaccattcttggcagcagctgagacagtctgagaacctgctggaggaaaagtaattccttcttctttcatagatttaatagttgcagatatcagactaaactgagggtccttctgaaattcttctgaccactccaccattaaagatttcagtttttcacatactttaggatgtgccttatttttaatcacagcacgtacttctgttgcaaaatcacgggaacatacttctaaatgaaatatctttccacagtttgccacacaagccccaagaagagttagtgcttgcagagcaacatgtggaaccttatgatttacccttttcattatggcttttaggcaatctttcgctccattaggagtacttccaactttgtcacatatgtccataataagactccaatcttctgtagtgttgtactcattcgtggctttttccacgtcttgctcgaaggggttggcggtgaacaaaggcatctcgccggcgcccgagccctagtcgctgctgtctagctgacactcagcaactgctacccgccgggtgacccgcggccgcggctccctagaccgctccgcttcggcctccgtccctgcactt

SEQ ID NO: 11114 - RNA, 3946 nt, Homo sapiens
  source 1..3946: mol_type = other RNA
ctgaatagctgggactacaggtgcataccaccacactagctaatttttttatttttatttttattaaagacaaggtctcactatgctgcccaggttggcctcccaaagtgttgggattacaagtgtgagtcaccgtgcctggtcccatgaactttaggtcatcactaataaaatgtatagatattgtatcatggcaacagttgttatactgtactttctaattgtatttttattgtttttttcttcaaatattcagccttatctagttgaatctgaagatgtggacctgctgatgaagagggctgactgtatctaacttagggtcttgcatgtagctggtacttaacgcattttattgactgttttagctaacattcaatggacaattcctaataaaaacctcttaaaagtatgaaaaaaaggaaacctgctctaaagtggcaggaaaaccagcctgggcaacatagcaagatcttgtctctacaccaaaagttttaaaattcactgcctgcctgtagtcccagccactcaggaagctgaggcaggaggatcccttaagcccaggagtttgaggttacagtgagctagatcacaccattgctctccagtctgggtgacaacaaggccctgagaaagaaaaaaaaaagaaaggaaaggaaggaaagagtgtaagtattgaaaaggaagagacaaaactataattatttgcatataaaataataaatgttagccaaagaagcctaagagaatcaactaagattttactggaagtaatatgagaattcagtacggtggctagaaacaaaatcaagagagcagcacacaaacctcaaatgcttttcagatgtaccaccaataactaactagaaaatggaagaaagatcccatttacaatggcaatacaaatgtctgaagtatttaggaacaaaaatacaaagatctgttatctaacaaaagacgtgtaagatctatatgatggaaaccctaaaactcttctgaaagacattaacaagaaatgaatacatgacatgaaataccatgttctagaatgtcgtacagatgtcaattctcaaattaatctacaaatttaaggtaatcctattcaaatcccaagatagtttttggtggtggctgtttttgagacaaggtctcgctctgttgcccaggctagagtgcagtggtatgaccacagctcactgcatcctcgacctcccaggctcaagcaatcctcccacttcagcctctgaagtctcttatatggtgtccaagaaatggggacaaatctcacaaagggactaggctcaggagggctggaatattcagggaagtttctttttttttttttttttgaggcagagtctcgctctgtcccccaggctggagtgcagcggcccgatcttggctggctgcatgctccacctcccaggttcatgccattttcctgcttcagcctcacaagtagctgggacgacacacgcccgccaccacacccagctaattttttgcatttttagtagagaatggtctgtgttagccaggatggtctcgatctcctgaccttgtgatccgcctgccttggcctcccaaagtgctgggattacaggcgtgagccaccgcacctggcctattcagggaaggtttcaagcagaaagatgaactgagttggctttggagagattcacaggactcccacaggcagagtgaaataagggcattgtagatggacaaaggcacagatgagcagcaatggggacagtgtgactgggggacgctgaggggctgctgtggctggaatggagggctgccaccataatggaaatggccaatgaggcaaataaggttggattaggagcatagcatcaagggtgccagcttattaaatccctcttccagtatgctagcactggcctgctgggaaaagtaatacatcacataatcaaacaaaaggcaaaaagaggcgagctccaggaataggcactgtaaacaggactcgccccagggtagccagatgcaggctttagatttgttgatgcaggttgagcatctctaatccgagggggaatgtctcatatggtgtccaagaaatggtgacacatctcacagagggcctaggctcaggagggctggagtatgagacattccccctcccctgtgaatttgaaaacgtggccaaaatttttttttaaaaatggctaccctgtagttctttaactggacctatttagacaacaccttacacactggagaaggatgatactatgtgaatctagtaagtctacaagacaatacttctctcttttggctgtcttcttcctctccagggtgatgacaactccgtgagggtggagattatatgtctctcatcatttaagcaacaaggaaataaattagtggcagagtaaggggtgactcagtgagtacatccaattgttgacatagttttgggtgggagaaattttgctattatatcaacttaacttcttaaaatagtctagtgggattaacttggttttatttcacagagacctcctggaagcgaggatcctttaacaatcctggaatatacattgcagtaaaagaacaaagcacacctcagccttaaatgacagaagaagaatgtcaagtgggaaagtgacgttggttttcagtttgtggattctgaatccacacaaacacaggattgtattttgaaaacctgaattaattattgtctttacctctataaaacaaaaaattataatcaaaattattagtatgacagtcacagatattgcgaagatgagtttgttcttatagtcatatcctggaacttctttcatgagctcacttgacttctgctctttctgttcattctgttccatgttctcattaatataatttgttttttgttggtccgtatcccattctacattcaatgcctttgcttcctgctgctcgctgagaagcttcatcaggaggcctgttcgcgacatgagcttggcacagctcccttgcacatgtgtttctgaacattccattttcaaggtccagataacatgagacatgaactttctcacatcctcgttggggatgagggaccgtagctgctcggttagctgaatttcaagctgatcacatcactctcgtcattggtgtctagctgctcactcccaaagcctgacaagttgatgccactgctgtctgagggcgcctccgactcaatagtcagctcagtgctcatgtgctgcttccgggcttgtaacatcttcatgaatgctccttctggattccctacagatgcttcttcagttgtctggtaaatcattatcaaataaatgactgcagtccacaacttgtcctcctgtgccgatttggtccctggactgaagacttactactgtcttctaactgtcctttggcccaagtttgcataaatccaacctctgataaccagtgtctttgaggtggttgatggcactggaaaaagacgaacacaacggagaaatccagcaccttgtttcttatggatcttcttgtgattccatacactgattgtaactgaatcagacttttcaatatacctattatattttaaaatgctgtagaacaaaagctgtttctaacgcttttcccctgcttctttcctgtatgcaggccttgaacgagcaggactcttgcagatttcacttcacctcctgggggaggcgatcgggttacctgccggctcctgctcttttcaggtgcagccaaggatagggagatgataacatcaggcccgagacgttgggagaatggagaagcgcttgcgagccaaaagtcctccaggagcacctgaaggaagcttcgcctgcacctgggacacccttccctgatgctggcctcaaggcaggcgcgccgcacacgcttccggtccatgacgaccacagctcagaagagcacgcgaacccagcctccacaaagagaaaat

SEQ ID NO: 11115 - RNA, 2285 nt, Homo sapiens
  source 1..2285: mol_type = other RNA
ctgaatagctgggactacaggtgcataccaccacgcctggctaatttttgtaatttttttcccaagatggaatcttgctctgctgcccaggctggagtgcagtggcatgatcttggctcactgcaacctccacctcccgggttcaagcaattctcctgcctcaggctcccgaatagctgagtttacaggtgcccgccaccacacccgattaatttttgtatttttagtagagacggggtttcaccatgttggccatctggtctcaaactcctcaggcgatccacccacctcggtctccctaagtgctggggattactggcatgagccaccgggcccggcttgacacaaccttttctgagggcagagatcagtcaggagtgtgactgcatactcagccaggaataagttacaaccttctcctgaaagcagcacacaggcagcagagtcacatcacctgggtgctgagcccagcaatcagtaacaatgctctctgtggtccaggcccaggcagcagagacacatcacctggtacctgggccagccacaattttttctgtggggcacgtacaggcaaaaatggagcatcacatctcctaggttattgatgcagaggtatgtcacaaggccctctgtagaaagagcccaggtggtagtctcccattttataggtgttggacctagtaatatgtcttaacatgaaaaatattcagggcctaagcaaaaaaggagagtcacataacctgagtgcagggcttaggaatatgtcacaatgcaacatgtgggcagctccaaggctggaaaaaagagtcacatcttggaggttcagagtcaagccatatgtcacaatctcatttgtgtgcttggccaaggcaggagagtcaaatcactaaggtgctttgcaatgcacacaatcacacctgcaggaaagtccagggattagattagaaattccaaacatgtccaggttctaaaggtatgaaagtcaacacctcctgtatgttgggtctaagtacatgagtcgcaatcacaatgattgacagaatgtgtgcaaaagagccacagtttcttctgcagactgtatcttcttagtgtagtcacagccttacatgtgcgctgaaccttggtctggaagtcactaacccacctgtggaccagatccacacatgagaggcaattatccaacttttgacagcctctgtgaaattcagaacttcaacagtgggatgtgtttatgtgggagaatgacaatctttactgttgcctgggtgtgcattcgagagacactctgtgtcacctgaggactttatacaatatgcaagattgataatcctctatgacctttgcacaaggagctccagaatctttcctgtggttctaagcccagatatgagagtcaacatctctctcaccaactgagtccagataggagagtcttcaccttcctatgagctggatttagaaatgagtcaccatcccaactgtagccagatgttcacatatgacagtcacaattccaactgcggactgtgttcacatgtaattcagaacctcactagcagactctgtcaatgggtcagggtgacaactgtaaaggttggtgtagtgtgcataggacaaacacaatctcacttgtgtgctgggccctgttatgacattctctgtaacacactagggcgtaatatatgtgagagagtagtaattctttatgacttttgtacagaaagacttcctcattttcctaagcctgagagcaacattctctctgctattggcttcttcaaggtatgacagtcatcattacatctgtacgcttggccagatatatgtcacaatcctacctaggtgctgggtccagtgatctgtcacaatcttttcttttggcaggcctgaagcagaagagtcacgttacatcatcttggtgctgggcacagcagtatgtctcaatgccttccaagggcacagccaaagcaaataactaacatcaccttagtgttaggcccagcaatatgtcacaatctcctttgttgtcagaacctgggaggcggaggttgtagtaagccgagattgggataatgcactccagcctgggcaacaagagtgaaactccatcttttcccagcttccaggatgtcctggcatcttagctgtgcgtctcccagaacctgcagatcacagggcaagaggctgtgacagtcaccgggggctcccgaggtggaggacgtaaaacagcagagaccgatcccaagctgtggcgggagtgagatacaaaggccccaccaaatgcc

SEQ ID NO: 11116 - RNA, 2210 nt, Homo sapiens
  source 1..2210: mol_type = other RNA
ctgaatagctgggactacaggtgcataccaccacgcctggctaatttttgtaatttttttcccaagatggaatcttgctctgctgcccaggctggagtgcagtggcatgatcttggctcactgcaacctccacctcccgggttcaagcaattctcctgcctcaggctcccgaatagctgagtttacaggtgcccgccaccacacccgattaatttttgtatttttagtagagacggggtttcaccatgttggccatctggtctcaaactcctcaggcgatccacccacctcggtctccctaagtgctggggattactggcatgagccaccgggcccggcttgacacaaccttttctgagggcagagatcagtcaggagtgtgactgcatactcagccaggaataagttacaaccttctcctgaaagcagcacacaggcagcagagtcacatcacctgggtgctgagcccagcaatcagtaacaatgctctctgtggtccaggcccaggcagcagagacacatcacctggtacctgggccagccacaattttttctgtggggcacgtacaggcaaaaatggagcatcacatctcctaggttattgatgcagaggtatgtcacaaggccctctgtagaaagagcccaggtggtagtctcccattttataggtgttggacctagtaatatgtcttaacatgaaaaatattcagggcctaagcaaaaaaggagagtcacataacctgagtgcagggcttaggaatatgtcacaatgcaacatgtgggcagctccaaggctggaaaaaagagtcacatcttggaggttcagagtcaagccatatgtcacaatctcatttgtgtgcttggccaaggcaggagagtcaaatcactaaggtgctttgcaatgcacacaatcacacctgcaggaaagtccagggattagattagaaattccaaacatgtccaggttctaaaggtatgaaagtcaacacctcctgtatgttgggtctaagtacatgagtcgcaatcacaatgattgacagaatgtgtgcaaaagagccacagtttcttctgcagactgtatcttcttagtgtagtcacagccttacatgtgcgctgaaccttggtctggaagtcactaacccacctgtggaccagatccacacatgagaggcaattatccaacttttgacagcctctgtgaaattcagaacttcaacagtgggatgtgtttatgtgggagaatgacaatctttactgttgcctgggtgtgcattcgagagacactctgtgtcacctgaggactttatacaatatgcaagattgataatcctctatgacctttgcacaaggagctccagaatctttcctgtggttctaagcccagatatgagagtcaacatctctctcaccaactgagtccagataggagagtcttcaccttcctatgagctggatttagaaatgagtcaccatcccaactgtagccagatgttcacatatgacagtcacaattccaactgcggactgtgttcacatgtaattcagaacctcactagcagactctgtcaatgggtcagggtgacaactgtaaaggttggtgtagtgtgcataggacaaacacaatctcacttgtgtgctgggccctgttatgacattctctgtaacacactagggcgtaatatatgtgagagagtagtaattctttatgacttttgtacagaaagacttcctcattttcctaagcctgagagcaacattctctctgctattggcttcttcaaggtatgacagtcatcattacatctgtacgcttggccagatatatgtcacaatcctacctaggtgctgggtccagtgatctgtcacaatcttttcttttggcaggcctgaagcagaagagtcacgttacatcatcttggtgctgggcacagcagtatgtctcaatgccttccaagggcacagccaaagcaaataactaacatcaccttagtgttaggcccagcaatatgtcacaatctcctttgttgtcagaaccttttcccagcttccaggatgtcctggcatcttagctgtgcgtctcccagaacctgcagatcacagggcaagaggctgtgacagtcaccgggggctcccgaggtggaggacgtaaaacagcagagaccgatcccaagctgtggcgggagtgagatacaaaggccccaccaaatgcc

SEQ ID NO: 11117 - RNA, 9088 nt, Homo sapiens
  source 1..9088: mol_type = other RNA
ctgaatagctgggactacaggtgcataccaccatgcacggctttttcttttagcttttggagagacaagtttccactatgttgcccagactggtctcaaacttctgggctcaagcaatactcctgccttgagctcccaaaatggtgggattacaggcataagctgccccctgcagccatattcttatcattactatttaaacgagtgaagaaagcatttttaaggttcctattccaaatttgcctaaaagatgaactccagcccaggggcaggagacctaggctggaaggcactgccggtcctagtccgctcctcctgggcccctgggtctgcggtgagcaggtggcagctctgttgtctccctcccccatctaggcgggcctggacgccaccccaatatcgcaggccacatagggctccacgcgctcctccctcttgctctgctcttccctcgggccctgtgggaattctcgagtcaagcccagccgcccctgctgacccaggtcaaggctctcacggagcatggggcctgcacgctttgaacctcttgaaacattataagcagaacattgccccacagcctgagagccacagccgtgtctctcctaagcaaggatggtgcttagacaaggaaaaaagacagggcctggctttttcatcctaggatttcaaagtgcatttagacacgctaacttatgaccactcacgaggtggtaacttcacacggccggagaaacgacagcacaagaagtatcgttgactcccgaccccaagataaatccagaatgacacaggattgtgcaacctccagatctttgttcaaacagcttattctaccagataaacctgagcggcggcattcttcttggcagtttctggaagtgtgaaggtgaattcctaactaagatagaaggtgactacaggtataaaccaccacctcccaaatcagcctgtagaccctccactgtgggtacctcgggctggccctacaggcccactctgtcttctcttcggtggcccaccccgctcctactcacaaccgagcctcatctggggtgcccagttcccatcatcccaggaaagtctgggaccctctgcctttcagagttcaggtcaaacactaccccaaagacctgagctagaattttcaagtccaaatctccaaacacacacacacacacattctcttgcacacaagtgcagactcacacttgcacgcacacttgcacatgcactcgcacacctgcacacacacaccccgccagcttctagccagtacttcaaacccccaaactataagtgcaaaaaacacccagataggctgtgttcgtttatcactgtcaaagtcaaccaacagatcctcatcagacaagtgtgacgggaccattacagtgagcaaatgctctccagatggcaccatgacagccatgggagtcatttcaggcatgcctgcggaatggtgcttggctcagatcagtagcgcccacggacagacacagagaagccttcaaaccaggtgtcctttcttcattagcctccccatcagagatgcactgagaaattattcctgctgggcacagcagcccacgcctgtaatcccagcactttgggaggctgaggcagaaggagcactcgagctcaggagtttgagaccagcctgggtgacaaagcaagaccccgtatctaccaaaaaaaaaaatttttttttgagacggagtctcgctctgtcgcccaggctggagtgtagtggcgccaatctccgctcactgcaagctccgcctcccgggttcacgccattctcctgcctcagcctcccgagtagctgggactacaggcgcccaccaccacgcccggctaatttttttgtattttagtagagacggggtttcaccatgttatccaggatggtcttgatctcctgacctcgtgatccacccacctcggcctcccaaagtgccgggattacaggcatgagccaccgtacccggcctctaccaaaaatgtaaaaattagccgggcatggtggtgcatgcctgtagtcccagctacttgggaggctgaggtgggaggaccacttgagcccaggaggtcgaggctgcagtgagctatgatcacaccactgcactccagcctggatgacagaaagaaactctgtcaaaaaaaaaaaagaacaaattatttccaaaggggaaaaaattacacattctccaattaatctctctgctggtgaaatggtatcccaataggagagcctcacctatccctgggtcctggcagagtaagaacatgtttctaaaatctcatgatgctaagaaacggctcatgtccacgtgaacagtgccctgcatcctcaggtcacgtggcttctctcttcactgatggaactccttcaaccctagtttatcaaacaccaacatattaatgcagttgtgtgcgagtctagatcctgtatgtgaaacgctagaaatccaacccaaatcagctgaagcgagtgcaaattcctggaggcgcacagctgagaagagcaggtggagccggcttcaggtgctcaccccggcccggcccccgatctggtggcccttcctccctcagcagttggtctcagttccgggacggcttttctaggtggccacagcactgtaacgtccatcccctccacctgccagaacctcttcccagaggctcacagctaagagcactgggtctcaggggtccaggtcaggaaatcagccccgtcccgtatcaaccatgggacacaatggctcaggtgcatctgcccttgggcctgggtagggaggcctgactcagccctcctagggtaagggagagggcggaagagacgggctctctgaccaggaggaggaatgcacacaggcaaaacacaacagatgtgtgcaaacagtcactccaacactcgggagaaacgtttaaagacttttaggttaattacgtccatgcaagccaagctttcccttttgatattcttaggtttggtaggatagaagaggatgtgtggcttataaataagtgagcaaaaattacccctggataatgggcatgggagcgccccagcctggtgatggcatccttgggggctgggtggtatctgcagcctgtgtgatatttgggagtctgttattcttcagggtggggctgccaatgagaacagagcgtccccagctctctgccaagagtctcagccgctcccctgggctgcctccatacaggcgggtgagcacacatggaggggagcaccaccaggaacccaggcttcctttcagagactctagggagaagactctggggacgttggtgtggccccaacattctgccgcagggaaacacctgtcaccatgccgaaccaacacattcaggaaaggtccccccaccaaggtacaaccaaggcagttcacatccagggacaggtgccccgggcagctcagctcaggagggtccctctggggagacctggtctgcaccaggaagcagaccacgtgttcacaaaatgcacacgccacccactttgcttggacccacacaaggaccatgtccacagcttccagctcagatggctgctcccatccgtgtcactgtccctcacagggacgagggcttagccaccctgcgttcactctccacccctacggcagccctgccagcctctcacctgagtgcaggagacagggcggggagagagaggtgcggccatccaggccccgatgaatgcagctggcctcatcggagggtttgcaggaacaaacttggaacacaactcctacaccctctggaagaaggaaacaagaaaaatatcccgatgtgtgtgtgagagagagtgtgtgtgtgtgtgtgtgtgtgcgcgcgtgtgtgtgtgtgttctgattcctaagtggcagagctaggttaaagccccaccttcaccaaaccacccacctcagggcacagacgtgctcagacctcaccgggaagataaactgaaatcctaacccttgccctccatcaagacatagggccaaaaccaaacctgaaatttttccaatagtccaaataaatggcaaaagcactacagcaaactccactaaatatccactgggggttgtaagtatcagcgaatgaagaagcatgagatgctttaagaggaaagagggagggaggcatcacccacacaacctgcaagtcacacctgtgtcaaattcctggggcagatggaaaatacacagcatcagacgctgggaggcgagtccaggagcagccaggccgcccagcccaagcattgcccaactgtaaacgggcgaggtgccctcccactgattcgaggcgcagccatcacacaagagacagggctttgtgacaccaccccgcacccaaccaagtcattctcatgactgtgctcaaagtgtggacacagctggaggatgggggccaacagggtaaaagagttttaagtttatggttaaattttccagttgtacgatgccaattttcataaaatgtataatttgctgtgtttcagtggaaaaagaaaaaaccagagccaaaggtctctacgcagtgtggtgctgcgcatcaggcaaacagcgaagaatcaaagtgggttctccccgctcacacctccctctcttcccggagacgcctcccctcggcccagcaggcccttttctgccactcccatccggagtcatccccacgggcggtggccccgaccatggcccgggaatctgagcaggtgcgtggatgtgggtggtgtcttctgcaggaacccctccacatccctgcaaacaccccaggtgctcaggaaaaccgaacctcagaggaaccataccaagaactgggaatgcagaaatggaggggacgcgggcccccctcagtgagtgaaccgcccagtgggttctgacattcgtctgaacatcctataaacaaacgcatcccggggaggtgctccagcaaaggcagacacaaagggccatgcccagaatacggaaaacaagccctcagcagattcactgacaccctgttcacagcagcattcaattcacattcgcaggaaggcagaagcaactcagtgtccaccaactgatgaacagataaacaaaccatgcctcttccacacaatgggacattattccgcctcagaaaggaagttagttctgacacctgccacgacaccgatgaacctagaggacattgcatgaggtgaagtacttcagtcccaaaaggaccaatactgtgtgactccatttctgagggagctcgggtagtagaaatcagagagtggaagctgctgccttctaccaatggggagcgagtgctgaatggggacagagtttcagtttgggaagatgagaaagctctggagatgatggtggtggtggcacgacaatacgaatgtgcttaatgccacacaacagtgcacttaacaatggttaagatggtacgtttaaaattaaacatttttatcataataaaaaacttggaggggccaggtgtgatggctcatgcctgtaatcccagcactttgggagggtgatgcaggagggtcacttgagcccaggagtttgagagcagcctgggcaacacagtgagacctcatctctgctgaaaataaaaaactagctgggcaggctggcgctcacctgtaaccccagctacttgggagtctgagatgggaagatcacttgagcccaggaggttgaagctgcagtgagctgtgattgcaccagtgtattccagcccggatgacagagcgagaccctgtctccaaaaacaaaacaaaacaaaaataaaagaaagcgaagcttcagaaaggaaggcaggaggtgtctaacacaggggacacctgaggctagcaggcactgggggccaagacccacacaagcccacctgagcctgggaaacacagggacaccacacacagaggacaccagggtatgtcccaactgagcgtggccagcaaccagggactgggcagtggtgacaaataccacacacgaggaagacaggtcaagcagggtgcccgacaccacgaaatgattgcaaccatctctccaactacagcttagaagcagaaatagcaaaggagtttcagccagatgtttccagagcctcctctgacacttttatcaagacagggcccatcaaacctgagggttcaaggtcagtcgtgtccttgagggtgaaggcactggagctaaaccaaccagaaagccacagagacagtcacacggagcctcttcttggtgacactgggtactgtcatccagcacggtctagagataaacgccaaaccactccactcctgccaactgtaaacctcaacagccatagtttactttctatttaatctatctatctacctatcttctatctgtctatttagaaacagagtctcactttgctgcccaggctggagtgcagtggcacgatcataggtcactgcagccttgaactcctgggctccagcgatcctcctgcctcagcctcccgagtagctgggattacaggtgtgcaccatcatgtccggctgattttcttattttttgtagacacagggtctcgctatgtggtccaaactgatcttgaactcctgggctcaagtgatcctccctcctcagcctcctgagtagctgggtttacagatgtgcaccaccacgtcctttttattttttgtagagatgaggtccttgctatgttgcccaagctggtcttgaactcctgggctcaagtgatcttcccccctcagcctcccaaagtgccaggattgcaggcatgagccaccgtgcccagccttaatagccataatgtattaatatttatttatttattttgagatggaatctcactctgtcacccaggctagagtgcaatgtcgcgatctcagctcactgcagcctctgcctcctgggttcaagcaatctttccatctcagaactcctgagtagctgggactacaggtgcacaccaccacacccgactcatttttttttttttttttttttttttttttttttttttagtagagacagggtttcaccatgttggccaggtctcaaattcctgacctcaagcgatccttctgtctgggcctcccaaagttctgggattacctgcctgagtcacccgcccggccttaacagccataatttaaactagacagtatgggaacagctggagttagaaatcctagaaatcctgcttctgtaactgaccggtttacctctgacttgacttcaaacaggaagccctgaagattgaccttttcaagtacaacacttaaacaaagaactttccctctggaaggatttgtcggctacccttccaaaaacagacaggtgcggcctgacttcaagtgcaggccccgccctcctccggtgagtggccctagccctggaggcagctccatcagcctcagcatcccctcccggcgcccgcacgctcagaaaaaccacaggagcgggcgagcgggcgagcgggcgggcgggtgggcgggcggaggggagaggggatattttactccagcattcccttccacatttcgtattaaatacctgaaatatattaatcttaaaaaacaatatcgatacagtactcaatggatagaggcagtggagtgaacaagaagcccagattgcaaaatcgtaggtcataaaaaaactggagtgcgcgtgcgtcaggttccaggcacgcgagaaaaagcaacgcgaaagctttcagtctcggaggaggttttcgggcttggggtagccgaagagaacaaagtcggcctcgtagagtttatacagctgctgcctccaggccagggggatcttggcgaaccagtcctcctcccagctgctggcggtcctgttccggtagctcggggggaagcggagctgccggtccacctggagtagctgcagcagctgcgcggcgtcctcgtccagagtctccagcttccccacgaagtcgtagtcgatctggcacgggtggcagaggcggtacacctgccgccagtgctcgttgaagggcgccagcttctccgtgtgcgggtccagcaggtactggatgaagttggcgaaggacaccttgaggccagcgcggaaggcctcgcgcgccgaggcgggcaggctggtgtggttggcgtacagccgcagcatgggcacggcgaacttgcggtagaactcctcgttctccagctcgaacttgctgcggaaggcggagatcaggcgcacgaaggggtcgcgcacgaagaggaacttggtgtacttcttgagcttgaccttcatgaggtggcgggagagcttcccgtagcggcgccagaacttgttgaaggtcaggtgcgcgctggcgttgtgcacgtgctcgcgcgggatgcgcagcgggtcgcggtagggcgcaccgcggtgcagcaggcttccgctcagcacgatcatcacgcgcttccagttggtgcaggccaccttgggcacgtagcagtagatggccccgtgccggtcgtccacgatcaggtggctcagctccgagttggggatgtcgtcgaatgcgcgctccttggtggggaaggccaggctggagttggcgcagaagccccgcagcacgctcctccgctccgcctgctgccggccctggtctgggctgcgccgggcgtcgcgcggggaccagtcgtagcctctcacgctctcctccatgctccccggcgcaggcggctgctccgtctcctttctgggaaggtcgctctgcttcacgccagcactgagaaacttgtccagaaactcgtcgacatcggagtcggccgtgagctccctgtccctgtccggcccgggcgtgggcagcggcggccccgtgtgcggcctagagaaggacgtgtgcaagtagaagtgcgcggcgcctgcgctgtcccagtacacgatgatcagcaggatcatgaacaccgaccccagcaccagccacagccggaacagccgggccttggtcatcctgccccgggcgggctgggccctctccgggcctctcacttcagcttcctgcagagccggggcatcctgctgggaacctcgcgaccctcacctcgcgcccctcacctcgcgcccgcagccgccgccgccgccccgcgact

SEQ ID NO: 11118 - RNA, 9074 nt, Homo sapiens
  source 1..9074: mol_type = other RNA
ctgaatagctgggactacaggtgcataccaccatgcacggctttttcttttagcttttggagagacaagtttccactatgttgcccagactggtctcaaacttctgggctcaagcaatactcctgccttgagctcccaaaatggtgggattacaggcataagctgccccctgcagccatattcttatcattactatttaaacgagtgaagaaagcatttttaaggttcctattccaaatttgcctaaaagatgaactccagcccaggggcaggagacctaggctggaaggcactgccggtcctagtccgctcctcctgggcccctgggtctgcggtgagcaggtggcagctctgttgtctccctcccccatctaggcgggcctggacgccaccccaatatcgcaggccacatagggctccacgcgctcctccctcttgctctgctcttccctcgggccctgtgggaattctcgagtcaagcccagccgcccctgctgacccaggtcaaggctctcacggagcatggggcctgcacgctttgaacctcttgaaacattataagcagaacattgccccacagcctgagagccacagccgtgtctctcctaagcaaggatggtgcttagacaaggaaaaaagacagggcctggctttttcatcctaggatttcaaagtgcatttagacacgctaacttatgaccactcacgaggtggtaacttcacacggccggagaaacgacagcacaagaagtatcgttgactcccgaccccaagataaatccagaatgacacaggattgtgcaacctccagatctttgttcaaacagcttattctaccagataaacctgagcggcggcattcttcttggcagtttctggaagtgtgaaggtgaattcctaactaagatagaaggtgactacaggtataaaccaccacctcccaaatcagcctgtagaccctccactgtgggtacctcgggctggccctacaggcccactctgtcttctcttcggtggcccaccccgctcctactcacaaccgagcctcatctggggtgcccagttcccatcatcccaggaaagtctgggaccctctgcctttcagagttcaggtcaaacactaccccaaagacctgagctagaattttcaagtccaaatctccaaacacacacacacacacattctcttgcacacaagtgcagactcacacttgcacgcacacttgcacatgcactcgcacacctgcacacacacaccccgccagcttctagccagtacttcaaacccccaaactataagtgcaaaaaacacccagataggctgtgttcgtttatcactgtcaaagtcaaccaacagatcctcatcagacaagtgtgacgggaccattacagtgagcaaatgctctccagatggcaccatgacagccatgggagtcatttcaggcatgcctgcggaatggtgcttggctcagatcagtagcgcccacggacagacacagagaagccttcaaaccaggtgtcctttcttcattagcctccccatcagagatgcactgagaaattattcctgctgggcacagcagcccacgcctgtaatcccagcactttgggaggctgaggcagaaggagcactcgagctcaggagtttgagaccagcctgggtgacaaagcaagaccccgtatctaccaaaaaaaaaaatttttttttgagacggagtctcgctctgtcgcccaggctggagtgtagtggcgccaatctccgctcactgcaagctccgcctcccgggttcacgccattctcctgcctcagcctcccgagtagctgggactacaggcgcccaccaccacgcccggctaatttttttgtattttagtagagacggggtttcaccatgttatccaggatggtcttgatctcctgacctcgtgatccacccacctcggcctcccaaagtgccgggattacaggcatgagccaccgtacccggcctctaccaaaaatgtaaaaattagccgggcatggtggtgcatgcctgtagtcccagctacttgggaggctgaggtgggaggaccacttgagcccaggaggtcgaggctgcagtgagctatgatcacaccactgcactccagcctggatgacagaaagaaactctgtcaaaaaaaaaaaagaacaaattatttccaaaggggaaaaaattacacattctccaattaatctctctgctggtgaaatggtatcccaataggagagcctcacctatccctgggtcctggcagagtaagaacatgtttctaaaatctcatgatgctaagaaacggctcatgtccacgtgaacagtgccctgcatcctcaggtcacgtggcttctctcttcactgatggaactccttcaaccctagtttatcaaacaccaacatattaatgcagttgtgtgcgagtctagatcctgtatgtgaaacgctagaaatccaacccaaatcagctgaagcgagtgcaaattcctggaggcgcacagctgagaagagcaggtggagccggcttcaggtgctcaccccggcccggcccccgatctggtggcccttcctccctcagcagttggtctcagttccgggacggcttttctaggtggccacagcactgtaacgtccatcccctccacctgccagaacctcttcccagaggctcacagctaagagcactgggtctcaggggtccaggtcaggaaatcagccccgtcccgtatcaaccatgggacacaatggctcaggtgcatctgcccttgggcctgggtagggaggcctgactcagccctcctagggtaagggagagggcggaagagacgggctctctgaccaggaggaggaatgcacacaggcaaaacacaacagatgtgtgcaaacagtcactccaacactcgggagaaacgtttaaagacttttaggttaattacgtccatgcaagccaagctttcccttttgatattcttaggtttggtaggatagaagaggatgtgtggcttataaataagtgagcaaaaattacccctggataatgggcatgggagcgccccagcctggtgatggcatccttgggggctgggtggtatctgcagcctgtgtgatatttgggagtctgttattcttcagggtggggctgccaatgagaacagagcgtccccagctctctgccaagagtctcagccgctcccctgggctgcctccatacaggcgggtgagcacacatggaggggagcaccaccaggaacccaggcttcctttcagagactctagggagaagactctggggacgttggtgtggccccaacattctgccgcagggaaacacctgtcaccatgccgaaccaacacattcaggaaaggtccccccaccaaggtacaaccaaggcagttcacatccagggacaggtgccccgggcagctcagctcaggagggtccctctggggagacctggtctgcaccaggaagcagaccacgtgttcacaaaatgcacacgccacccactttgcttggacccacacaaggaccatgtccacagcttccagctcagatggctgctcccatccgtgtcactgtccctcacagggacgagggcttagccaccctgcgttcactctccacccctacggcagccctgccagcctctcacctgagtgcaggagacagggcggggagagagaggtgcggccatccaggccccgatgaatgcagctggcctcatcggagggtttgcaggaacaaacttggaacacaactcctacaccctctggaagaaggaaacaagaaaaatatcccgatgtgtgtgtgagagagagtgtgtgtgtgtgtgtgtgtgtgcgcgcgtgtgtgtgtgtgttctgattcctaagtggcagagctaggttaaagccccaccttcaccaaaccacccacctcagggcacagacgtgctcagacctcaccgggaagataaactgaaatcctaacccttgccctccatcaagacatagggccaaaaccaaacctgaaatttttccaatagtccaaataaatggcaaaagcactacagcaaactccactaaatatccactgggggttgtaagtatcagcgaatgaagaagcatgagatgctttaagaggaaagagggagggaggcatcacccacacaacctgcaagtcacacctgtgtcaaattcctggggcagatggaaaatacacagcatcagacgctgggaggcgagtccaggagcagccaggccgcccagcccaagcattgcccaactgtaaacgggcgaggtgccctcccactgattcgaggcgcagccatcacacaagagacagggctttgtgacaccaccccgcacccaaccaagtcattctcatgactgtgctcaaagtgtggacacagctggaggatgggggccaacagggtaaaagagttttaagtttatggttaaattttccagttgtacgatgccaattttcataaaatgtataatttgctgtgtttcagtggaaaaagaaaaaaccagagccaaaggtctctacgcagtgtggtgctgcgcatcaggcaaacagcgaagaatcaaagtgggttctccccgctcacacctccctctcttcccggagacgcctcccctcggcccagcaggcccttttctgccactcccatccggagtcatccccacgggcggtggccccgaccatggcccgggaatctgagcaggtgcgtggatgtgggtggtgtcttctgcaggaacccctccacatccctgcaaacaccccaggtgctcaggaaaaccgaacctcagaggaaccataccaagaactgggaatgcagaaatggaggggacgcgggcccccctcagtgagtgaaccgcccagtgggttctgacattcgtctgaacatcctataaacaaacgcatcccggggaggtgctccagcaaaggcagacacaaagggccatgcccagaatacggaaaacaagccctcagcagattcactgacaccctgttcacagcagcattcaattcacattcgcaggaaggcagaagcaactcagtgtccaccaactgatgaacagataaacaaaccatgcctcttccacacaatgggacattattccgcctcagaaaggaagttagttctgacacctgccacgacaccgatgaacctagaggacattgcatgaggtgaagtacttcagtcccaaaaggaccaatactgtgtgactccatttctgagggagctcgggtagtagaaatcagagagtggaagctgctgccttctaccaatggggagcgagtgctgaatggggacagagtttcagtttgggaagatgagaaagctctggagatgatggtggtggtggcacgacaatacgaatgtgcttaatgccacacaacagtgcacttaacaatggttaagatggtacgtttaaaattaaacatttttatcataataaaaaacttggaggggccaggtgtgatggctcatgcctgtaatcccagcactttgggagggtgatgcaggagggtcacttgagcccaggagtttgagagcagcctgggcaacacagtgagacctcatctctgctgaaaataaaaaactagctgggcaggctggcgctcacctgtaaccccagctacttgggagtctgagatgggaagatcacttgagcccaggaggttgaagctgcagtgagctgtgattgcaccagtgtattccagcccggatgacagagcgagaccctgtctccaaaaacaaaacaaaacaaaaataaaagaaagcgaagcttcagaaaggaaggcaggaggtgtctaacacaggggacacctgaggctagcaggcactgggggccaagacccacacaagcccacctgagcctgggaaacacagggacaccacacacagaggacaccagggtatgtcccaactgagcgtggccagcaaccagggactgggcagtggtgacaaataccacacacgaggaagacaggtcaagcagggtgcccgacaccacgaaatgattgcaaccatctctccaactacagcttagaagcagaaatagcaaaggagtttcagccagatgtttccagagcctcctctgacacttttatcaagacagggcccatcaaacctgagggttcaaggtcagtcgtgtccttgagggtgaaggcactggagctaaaccaaccagaaagccacagagacagtcacacggagcctcttcttggtgacactgggtactgtcatccagcacggtctagagataaacgccaaaccactccactcctgccaactgtaaacctcaacagccatagtttactttctatttaatctatctatctacctatcttctatctgtctatttagaaacagagtctcactttgctgcccaggctggagtgcagtggcacgatcataggtcactgcagccttgaactcctgggctccagcgatcctcctgcctcagcctcccgagtagctgggattacaggtgtgcaccatcatgtccggctgattttcttattttttgtagacacagggtctcgctatgtggtccaaactgatcttgaactcctgggctcaagtgatcctccctcctcagcctcctgagtagctgggtttacagatgtgcaccaccacgtcctttttattttttgtagagatgaggtccttgctatgttgcccaagctggtcttgaactcctgggctcaagtgatcttcccccctcagcctcccaaagtgccaggattgcaggcatgagccaccgtgcccagccttaatagccataatgtattaatatttatttatttattttgagatggaatctcactctgtcacccaggctagagtgcaatgtcgcgatctcagctcactgcagcctctgcctcctgggttcaagcaatctttccatctcagaactcctgagtagctgggactacaggtgcacaccaccacacccgactcatttttttttttttttttttttttttttttttttttttagtagagacagggtttcaccatgttggccaggtctcaaattcctgacctcaagcgatccttctgtctgggcctcccaaagttctgggattacctgcctgagtcacccgcccggccttaacagccataatttaaactagacagtatgggaacagctggagttagaaatcctagaaatcctgcttctgtaactgaccggtttacctctgacttgacttcaaacaggaagccctgaagattgaccttttcaagtacaacacttaaacaaagaactttccctctggaaggatttgtcggctacccttccaaaaacagacaggtgcggcctgacttcaagtgcaggccccgccctcctccggtgagtggccctagccctggaggcagctccatcagcctcagcatcccctcccggcgcccgcacgctcagaaaaaccacaggagcgggcgagcgggcgagcgggcgggcgggtgggcgggcggaggggagaggggatattttactccagcattcccttccacatttcgtattaaatacctgaaatatattaatcttaaaaaacaatatcgatacagtactcaatggatagaggcagtggagtgaacaagaagcccagattgcaaaatcgtaggtcataaaaaaactggagtgcgcgtgcgtcaggttccaggcacgcgagaaaaagcaacgcgaaagctttcagtctcggaggaggttttcgggcttggggtagccgaagagaacaaagtcggcctcgtagagtttatacagctgctgcctccaggccagggggatcttggcgaaccagtcctcctcccagctgctggcggtcctgttccggtagctcggggggaagcggagctgccggtccacctggagtagctgcagcagctgcgcggcgtcctcgtccagagtctccagcttccccacgaagtcgtagtcgatctggcacgggtggcagaggcggtacacctgccgccagtgctcgttgaagggcgccagcttctccgtgtgcgggtccagcaggtactggatgaagttggcgaaggacaccttgaggccagcgcggaaggcctcgcgcgccgaggcgggcaggctggtgtggttggcgtacagccgcagcatgggcacggcgaacttgcggtagaactcctcgttctccagctcgaacttgctgcggaaggcggagatcaggcgcacgaaggggtcgcgcacgaagaggaacttggtgtacttcttgagcttgaccttcatgaggtggcgggagagcttcccgtagcggcgccagaacttgttgaaggtcaggtgcgcgctggcgttgtgcacgtgctcgcgcgggatgcgcagcgggtcgcggtagggcgcaccgcggtgcagcaggcttccgctcagcacgatcatcacgcgcttccagttggtgcaggccaccttgggcacgtagcagtagatggccccgtgccggtcgtccacgatcaggtggctcagctccgagttggggatgtcgtcgaatgcgcgctccttggtggggaaggccaggctggagttggcgcagaagccccgcagcacgctcctccgctccgcctgctgccggccctggtctgggctgcgccgggcgtcgcgcggggaccagtcgtagcctctcacgctctcctccatgctccccggcgcaggcggctgctccgtctcctttctgggaaggtcgctctgcttcacgccagcactgagaaacttgtccagaaactcgtcgacatcggagtcggccgtgagctccctgtccctgtccggcccgggcgtgggcagcggcggccccgtgtgcggcctagagaaggacgtgtgcaagtagaagtgcgcggcgcctgcgctgtcccagtacacgatgatcagcaggatcatgaacaccgaccccagcaccagccacagccggaacagccgggccttggtcatcctgccccgggcgggctgggccctctccgggcctctcacttcagcttcctgcagagccggggcatcctgctgggaacctcgcgcccctcacctcgcgcccgcagccgccgccgccgccccgcgact

SEQ ID NO: 11119 - RNA, 9060 nt, Homo sapiens
  source 1..9060: mol_type = other RNA
ctgaatagctgggactacaggtgcataccaccatgcacggctttttcttttagcttttggagagacaagtttccactatgttgcccagactggtctcaaacttctgggctcaagcaatactcctgccttgagctcccaaaatggtgggattacaggcataagctgccccctgcagccatattcttatcattactatttaaacgagtgaagaaagcatttttaaggttcctattccaaatttgcctaaaagatgaactccagcccaggggcaggagacctaggctggaaggcactgccggtcctagtccgctcctcctgggcccctgggtctgcggtgagcaggtggcagctctgttgtctccctcccccatctaggcgggcctggacgccaccccaatatcgcaggccacatagggctccacgcgctcctccctcttgctctgctcttccctcgggccctgtgggaattctcgagtcaagcccagccgcccctgctgacccaggtcaaggctctcacggagcatggggcctgcacgctttgaacctcttgaaacattataagcagaacattgccccacagcctgagagccacagccgtgtctctcctaagcaaggatggtgcttagacaaggaaaaaagacagggcctggctttttcatcctaggatttcaaagtgcatttagacacgctaacttatgaccactcacgaggtggtaacttcacacggccggagaaacgacagcacaagaagtatcgttgactcccgaccccaagataaatccagaatgacacaggattgtgcaacctccagatctttgttcaaacagcttattctaccagataaacctgagcggcggcattcttcttggcagtttctggaagtgtgaaggtgaattcctaactaagatagaaggtgactacaggtataaaccaccacctcccaaatcagcctgtagaccctccactgtgggtacctcgggctggccctacaggcccactctgtcttctcttcggtggcccaccccgctcctactcacaaccgagcctcatctggggtgcccagttcccatcatcccaggaaagtctgggaccctctgcctttcagagttcaggtcaaacactaccccaaagacctgagctagaattttcaagtccaaatctccaaacacacacacacacacattctcttgcacacaagtgcagactcacacttgcacgcacacttgcacatgcactcgcacacctgcacacacacaccccgccagcttctagccagtacttcaaacccccaaactataagtgcaaaaaacacccagataggctgtgttcgtttatcactgtcaaagtcaaccaacagatcctcatcagacaagtgtgacgggaccattacagtgagcaaatgctctccagatggcaccatgacagccatgggagtcatttcaggcatgcctgcggaatggtgcttggctcagatcagtagcgcccacggacagacacagagaagccttcaaaccaggtgtcctttcttcattagcctccccatcagagatgcactgagaaattattcctgctgggcacagcagcccacgcctgtaatcccagcactttgggaggctgaggcagaaggagcactcgagctcaggagtttgagaccagcctgggtgacaaagcaagaccccgtatctaccaaaaaaaaaaatttttttttgagacggagtctcgctctgtcgcccaggctggagtgtagtggcgccaatctccgctcactgcaagctccgcctcccgggttcacgccattctcctgcctcagcctcccgagtagctgggactacaggcgcccaccaccacgcccggctaatttttttgtattttagtagagacggggtttcaccatgttatccaggatggtcttgatctcctgacctcgtgatccacccacctcggcctcccaaagtgccgggattacaggcatgagccaccgtacccggcctctaccaaaaatgtaaaaattagccgggcatggtggtgcatgcctgtagtcccagctacttgggaggctgaggtgggaggaccacttgagcccaggaggtcgaggctgcagtgagctatgatcacaccactgcactccagcctggatgacagaaagaaactctgtcaaaaaaaaaaaagaacaaattatttccaaaggggaaaaaattacacattctccaattaatctctctgctggtgaaatggtatcccaataggagagcctcacctatccctgggtcctggcagagtaagaacatgtttctaaaatctcatgatgctaagaaacggctcatgtccacgtgaacagtgccctgcatcctcaggtcacgtggcttctctcttcactgatggaactccttcaaccctagtttatcaaacaccaacatattaatgcagttgtgtgcgagtctagatcctgtatgtgaaacgctagaaatccaacccaaatcagctgaagcgagtgcaaattcctggaggcgcacagctgagaagagcaggtggagccggcttcaggtgctcaccccggcccggcccccgatctggtggcccttcctccctcagcagttggtctcagttccgggacggcttttctaggtggccacagcactgtaacgtccatcccctccacctgccagaacctcttcccagaggctcacagctaagagcactgggtctcaggggtccaggtcaggaaatcagccccgtcccgtatcaaccatgggacacaatggctcaggtgcatctgcccttgggcctgggtagggaggcctgactcagccctcctagggtaagggagagggcggaagagacgggctctctgaccaggaggaggaatgcacacaggcaaaacacaacagatgtgtgcaaacagtcactccaacactcgggagaaacgtttaaagacttttaggttaattacgtccatgcaagccaagctttcccttttgatattcttaggtttggtaggatagaagaggatgtgtggcttataaataagtgagcaaaaattacccctggataatgggcatgggagcgccccagcctggtgatggcatccttgggggctgggtggtatctgcagcctgtgtgatatttgggagtctgttattcttcagggtggggctgccaatgagaacagagcgtccccagctctctgccaagagtctcagccgctcccctgggctgcctccatacaggcgggtgagcacacatggaggggagcaccaccaggaacccaggcttcctttcagagactctagggagaagactctggggacgttggtgtggccccaacattctgccgcagggaaacacctgtcaccatgccgaaccaacacattcaggaaaggtccccccaccaaggtacaaccaaggcagttcacatccagggacaggtgccccgggcagctcagctcaggagggtccctctggggagacctggtctgcaccaggaagcagaccacgtgttcacaaaatgcacacgccacccactttgcttggacccacacaaggaccatgtccacagcttccagctcagatggctgctcccatccgtgtcactgtccctcacagggacgagggcttagccaccctgcgttcactctccacccctacggcagccctgccagcctctcacctgagtgcaggagacagggcggggagagagaggtgcggccatccaggccccgatgaatgcagctggcctcatcggagggtttgcaggaacaaacttggaacacaactcctacaccctctggaagaaggaaacaagaaaaatatcccgatgtgtgtgtgagagagagtgtgtgtgtgtgtgtgtgtgtgcgcgcgtgtgtgtgtgtgttctgattcctaagtggcagagctaggttaaagccccaccttcaccaaaccacccacctcagggcacagacgtgctcagacctcaccgggaagataaactgaaatcctaacccttgccctccatcaagacatagggccaaaaccaaacctgaaatttttccaatagtccaaataaatggcaaaagcactacagcaaactccactaaatatccactgggggttgtaagtatcagcgaatgaagaagcatgagatgctttaagaggaaagagggagggaggcatcacccacacaacctgcaagtcacacctgtgtcaaattcctggggcagatggaaaatacacagcatcagacgctgggaggcgagtccaggagcagccaggccgcccagcccaagcattgcccaactgtaaacgggcgaggtgccctcccactgattcgaggcgcagccatcacacaagagacagggctttgtgacaccaccccgcacccaaccaagtcattctcatgactgtgctcaaagtgtggacacagctggaggatgggggccaacagggtaaaagagttttaagtttatggttaaattttccagttgtacgatgccaattttcataaaatgtataatttgctgtgtttcagtggaaaaagaaaaaaccagagccaaaggtctctacgcagtgtggtgctgcgcatcaggcaaacagcgaagaatcaaagtgggttctccccgctcacacctccctctcttcccggagacgcctcccctcggcccagcaggcccttttctgccactcccatccggagtcatccccacgggcggtggccccgaccatggcccgggaatctgagcaggtgcgtggatgtgggtggtgtcttctgcaggaacccctccacatccctgcaaacaccccaggtgctcaggaaaaccgaacctcagaggaaccataccaagaactgggaatgcagaaatggaggggacgcgggcccccctcagtgagtgaaccgcccagtgggttctgacattcgtctgaacatcctataaacaaacgcatcccggggaggtgctccagcaaaggcagacacaaagggccatgcccagaatacggaaaacaagccctcagcagattcactgacaccctgttcacagcagcattcaattcacattcgcaggaaggcagaagcaactcagtgtccaccaactgatgaacagataaacaaaccatgcctcttccacacaatgggacattattccgcctcagaaaggaagttagttctgacacctgccacgacaccgatgaacctagaggacattgcatgaggtgaagtacttcagtcccaaaaggaccaatactgtgtgactccatttctgagggagctcgggtagtagaaatcagagagtggaagctgctgccttctaccaatggggagcgagtgctgaatggggacagagtttcagtttgggaagatgagaaagctctggagatgatggtggtggtggcacgacaatacgaatgtgcttaatgccacacaacagtgcacttaacaatggttaagatggtacgtttaaaattaaacatttttatcataataaaaaacttggaggggccaggtgtgatggctcatgcctgtaatcccagcactttgggagggtgatgcaggagggtcacttgagcccaggagtttgagagcagcctgggcaacacagtgagacctcatctctgctgaaaataaaaaactagctgggcaggctggcgctcacctgtaaccccagctacttgggagtctgagatgggaagatcacttgagcccaggaggttgaagctgcagtgagctgtgattgcaccagtgtattccagcccggatgacagagcgagaccctgtctccaaaaacaaaacaaaacaaaaataaaagaaagcgaagcttcagaaaggaaggcaggaggtgtctaacacaggggacacctgaggctagcaggcactgggggccaagacccacacaagcccacctgagcctgggaaacacagggacaccacacacagaggacaccagggtatgtcccaactgagcgtggccagcaaccagggactgggcagtggtgacaaataccacacacgaggaagacaggtcaagcagggtgcccgacaccacgaaatgattgcaaccatctctccaactacagcttagaagcagaaatagcaaaggagtttcagccagatgtttccagagcctcctctgacacttttatcaagacagggcccatcaaacctgagggttcaaggtcagtcgtgtccttgagggtgaaggcactggagctaaaccaaccagaaagccacagagacagtcacacggagcctcttcttggtgacactgggtactgtcatccagcacggtctagagataaacgccaaaccactccactcctgccaactgtaaacctcaacagccatagtttactttctatttaatctatctatctacctatcttctatctgtctatttagaaacagagtctcactttgctgcccaggctggagtgcagtggcacgatcataggtcactgcagccttgaactcctgggctccagcgatcctcctgcctcagcctcccgagtagctgggattacaggtgtgcaccatcatgtccggctgattttcttattttttgtagacacagggtctcgctatgtggtccaaactgatcttgaactcctgggctcaagtgatcctccctcctcagcctcctgagtagctgggtttacagatgtgcaccaccacgtcctttttattttttgtagagatgaggtccttgctatgttgcccaagctggtcttgaactcctgggctcaagtgatcttcccccctcagcctcccaaagtgccaggattgcaggcatgagccaccgtgcccagccttaatagccataatgtattaatatttatttatttattttgagatggaatctcactctgtcacccaggctagagtgcaatgtcgcgatctcagctcactgcagcctctgcctcctgggttcaagcaatctttccatctcagaactcctgagtagctgggactacaggtgcacaccaccacacccgactcatttttttttttttttttttttttttttttttttttttagtagagacagggtttcaccatgttggccaggtctcaaattcctgacctcaagcgatccttctgtctgggcctcccaaagttctgggattacctgcctgagtcacccgcccggccttaacagccataatttaaactagacagtatgggaacagctggagttagaaatcctagaaatcctgcttctgtaactgaccggtttacctctgacttgacttcaaacaggaagccctgaagattgaccttttcaagtacaacacttaaacaaagaactttccctctggaaggatttgtcggctacccttccaaaaacagacaggtgcggcctgacttcaagtgcaggccccgccctcctccggtgagtggccctagccctggaggcagctccatcagcctcagcatcccctcccggcgcccgcacgctcagaaaaaccacaggagcgggcgagcgggcgagcgggcgggcgggtgggcgggcggaggggagaggggatattttactccagcattcccttccacatttcgtattaaatacctgaaatatattaatcttaaaaaacaatatcgatacagtactcaatggatagaggcagtggagtgaacaagaagcccagattgcaaaatcgtaggtcataaaaaaactggagtgcgcgtgcgtcaggttccaggcacgcgagaaaaagcaacgcgaaagctttcagtctcggaggaggttttcgggcttggggtagccgaagagaacaaagtcggcctcgtagagtttatacagctgctgcctccaggccagggggatcttggcgaaccagtcctcctcccagctgctggcggtcctgttccggtagctcggggggaagcggagctgccggtccacctggagtagctgcagcagctgcgcggcgtcctcgtccagagtctccagcttccccacgaagtcgtagtcgatctggcacgggtggcagaggcggtacacctgccgccagtgctcgttgaagggcgccagcttctccgtgtgcgggtccagcaggtactggatgaagttggcgaaggacaccttgaggccagcgcggaaggcctcgcgcgccgaggcgggcaggctggtgtggttggcgtacagccgcagcatgggcacggcgaacttgcggtagaactcctcgttctccagctcgaacttgctgcggaaggcggagatcaggcgcacgaaggggtcgcgcacgaagaggaacttggtgtacttcttgagcttgaccttcatgaggtggcgggagagcttcccgtagcggcgccagaacttgttgaaggtcaggtgcgcgctggcgttgtgcacgtgctcgcgcgggatgcgcagcgggtcgcggtagggcgcaccgcggtgcagcaggcttccgctcagcacgatcatcacgcgcttccagttggtgcaggccaccttgggcacgtagcagtagatggccccgtgccggtcgtccacgatcaggtggctcagctccgagttggggatgtcgtcgaatgcgcgctccttggtggggaaggccaggctggagttggcgcagaagccccgcagcacgctcctccgctccgcctgctgccggccctggtctgggctgcgccgggcgtcgcgcggggaccagtcgtagcctctcacgctctcctccatgctccccggcgcaggcggctgctccgtctcctttctgggaaggtcgctctgcttcacgccagcactgagaaacttgtccagaaactcgtcgacatcggagtcggccgtgagctccctgtccctgtccggcccgggcgtgggcagcggcggccccgtgtgcggcctagagaaggacgtgtgcaagtagaagtgcgcggcgcctgcgctgtcccagtacacgatgatcagcaggatcatgaacaccgaccccagcaccagccacagccggaacagccgggccttggtcatcctgccccgggcgggctgggccctctccgggcctctcacttcagcttcctgcagagccggggcatcctgctgggaacctcgcgcccgcagccgccgccgccgccccgcgact

SEQ ID NO: 11120 - RNA, 3223 nt, Homo sapiens
  source 1..3223: mol_type = other RNA
ctgaatagctgggactacaggtgcataccaccatgcctgacttattttttttccttttttttttttttttttttttttgatagaaacagggtttcaccttgttgcccaggctggtctcaaactcctggactcaggcgattcaccagcctcagcctcccacagtgctggggttacaggagtgagccaccatgcccagttaaaaatacactttttatttaaaaaaaaaagagaacactccttatatttcctttatattttgtaaactacatacccaaaataaagcatatcaaaaactgtaaaaaaaaaaaaaaaaaaccctaatatcagatattccagacacaacaataccataatttaatcacttaaaatcttactcaaaactaaatcaatgatcttttaggccaggtgtggtggctcatgatagtaatcacagtactttgggaggccaaggcaggaggatcacttgaggtcaggagttcaagaccagcatggccaacacaatgaaaatccatctctactaaaaatacaaaaattagccaggctaatggcacactcctgtaataccagctacttaggaggctgaggcaggagaatcgcttgaacctgggaggcagaggttgcagtgagccgagatcatgccactgcactccaggctggacaacagagcaagactccgcatcaaaaaaaaaaaaaagatattttaatatattcagatacacaaatatgaaataaaactaagtagagctggtattcatttacacataattatcttataccgtttggaataagaatttggggcacgttagcaaaccaaaaggctcagaaagacgtcgtgatatttagttcttgtctccctctacaaatgtgaagcactcttctatccggcattcctagtggagttcctattttcaaatttgcaaatcattctggtgctaagcaatctcaaaaaaaacatttactaaaaaccagaggaaaaaaatcttataactttgggaggctgaggcagatggatcactgagatcaggagtttgagaccagcttggccaacatgatgaaaccccatcttctctaaaaatacaaaaagttagctgggtgtggtggcaggtgcctgtagtcccagctattccagaggctgaggcaggagaatcacttgaacctctgaggcggaggttgcagtgagctgagatcgcgccattgcactccagcctgggcaacagagtgagactctgtctcaaaaaataaatataaaaaaataaaaagctgctattctccattaatacctgcaggcccgacaaaggcagcctaggaattctagatgaatggaatgaatacaacttgctggaagttcttaggaaacaaaatgactattcacagaaccaaataaaagccttccactagaaactaaaaataataataataataataatggttttatatatatgcatacacaagcaaagccagaagagaataaatagcaaatgaatgaaaactagaagcaaaaacaaacaggaaaccatctctacattttttttactcaatcgaccctgaatgctacagcattatccagggccgcagaaaacacacataatactttattcctgataaacaattcgatgtccttaagtccgccaatatcaccgtacattctgtgcaatcaagaaatttactcagctgggcacagtggctcacacctgtaattccagcactttgggaggccaaggcgggtggatcacctgaggtcaggcattcgagaacagcctggcccacatggcgaaaccccatctctactaaaaatacaaaaattagcccggtatggaggcatgtgcctgtaatcccagctacttgggaggctgaggcaggagaatggattgaacccaggaggcagaggttgcagtgagccaagattgcaccattgcactccagcctgggcaacagaacaagactccatcaaaaaaaaaaaaaaaaaaaaaagaaagaaagaagaaaagaaaattagccaggtgtggttgcatgcacctgtagtcccagcactttgggaggccaaggcaggaggatcaatcaaggctaggagtttgagactgcagaaagaaaccctgtctctaaaaaaaaggtccaggtaatttcagggtccagctccaccacaagcgcagctccaggggctgttgagttttgcctttatcattccaagtagtccctgctccagaccaagtcccaccatctggcagtcaggtcagtccaaccacagtcatatcagggcccttccaggaattctcgacgcaaactggaggccgatggcgcgggtcttttcgtggacggcggcagcacggtcctcggcttgcgtccgtagttgctcaggcttctggttcagggctgggcggcggcgcccctgcggcgggcggcccgcaccaggctctgctgcagcacggggtagaggcgctggcagccctcgaggcccaggcgtacggcctccgcccagctctctgtcaggccgccctcgccgctgcccagcagcccggccacctgattcagcacaggcatgagcgccacggtgaggccggcggcggcgcgctcttcctcgagccgcgtggggtccaggagccaggtgggcgcgggccccggcgcgaggctgaggccgcagcccaccaccaggtcgtacatctccacgcccgcgtcggccagggcgagcgcggcggcggtgagcgcggcggccagggccgagccaccgtcctccagcagcagcgccgacacctcgagctgcgcgcgcgggtagcggcccaggcgcacagccggctccagcgcctcctgcagcgccagcgccagctcacgctcctcgcagccgcccgggggagcgcggcgccggcggcccgcgaagggtgcgcggcggaagtcgcagagcaggcgaccgcgcagcgcggccggggcctcgccgcctgctccggccgggccgccgccgcgctcgccgccctcggcctgtcgcgggcccgacacggcacacagcaccttggtgcctcccgcctccaggtaggccgagcccttggcctggctcagcagcccggcgcgcgcgtacacgggccgtagccgcgttgggtcgcgggtgccgggcgcctcctcctcgtcggccgcgtacagctgcggcggctgcgattcttcagggccgcggatgcggcggtgatccccaggcatggcggttcttggcgtgcgaaccccttccgcccaacgccct

SEQ ID NO: 11121 - RNA, 1336 nt, Homo sapiens
  source 1..1336: mol_type = other RNA
ctgaatagctgggactacaggtgcatgccaacacggccagctaatatttgtatttttagtagagacggggtttcaccatgttggccaggatgttctcgatctcttgacctcgtgatctgcccacgtcagtctccgaaagtgctgagattacaggtgtgagccaccgcacccagcccacagcccacttttaacccacaggagctgatctgctgtcctgtccgctgcagtgcatggacttttttctcagcccttattttcccctattactgtgattttctccaagctgtcttccccatgtgctcatgaattccgggagatgacggataatccctgactcatccttgcaaccctgacacaacgcccaggccctgacatggagaagtgtccatgaagtctggttgaataaatgagtgaatgaatgaatgaatgaacaaaattagctagatgtagtgaggcctcttccaccaaaccacagctgaagggttttggagaaagcctcattctgcaaggaggtctagatctttattaggcctggccattggcggggcttgaacctcagagcccaccactcctagcacctcttcccctctcttctgctgtgcttcaaatggacccagagatgaattaagtcagagaaattcccaagtctcctttctatccacatccaggttaacattgctggaaagtgttttgcctactgaggacttctccttcccaatatgattcttggtatgtgctcacattgacttcgtattgagggcactgcattttattcaatgcgacagcatagcacagtgggtacatgcataggctgcagagtctgactacatttgttcaaatccagcttgaaccacttctcagttgcatggcatcaaatgtgttgttcgaccttgtgaaggctcagcttccttgtatttcagtgttatttaccagcaggaaaagacgattttgactgattgagttgaatgtgctgagttgatggtgagttcaatatggctgtaaagctcggtactgtcctggtcattgtgccttccgggagagggagaacgactgtgagttcctgagcccaaaggtgatcttttcttgctttgtagttctgaggagactgcacctggacaagttgtagaaatttgggctgtgcggtatgagatgcatgtatgcagactaaaaggcattcagccaacggatctgcatttggtaagagccggggattgggacgaggcagagagcaagaccaagctggtttcctctccggtttcctccggggtggctgggtcccaggtcctgcccccgcctcgccctgtgcaagctcggtgcagtgcagcccctccggctc

SEQ ID NO: 11122 - RNA, 1524 nt, Homo sapiens
  source 1..1524: mol_type = other RNA
ctgaatagctgggactacaggtgcatgccaacatgcccagctaatttttttgtatttttttgtattttttaatagagatagggtttcaccaggttggccaggctggtgtcacaactcttgacctcaagtgatctaccacccttggcctcccaaagtgctgggattataggcgtgagccactgtgcccggccaacattaatattttttattagctactacagcttagagtagctgctatgggagtgtggcctttttgattaaatactagctgatcaaccctagaatataaattcttgttttataacatttagatttaaataacaataagaatgtaagctccatgaaggcaagaatgcctttttgttttgttcactgctgtgtctaaaataatgcctggctcaaatatttgttgaatgagtaaatatgctgactttgctgaagtatttaagcaagttacagatattatacaagtaaatattttgggcacaagcacacttaatgaaacagtaaaaaaaaaataggtttgaaacacataatccttcgttataggaggctcaagagtttaaaaggaaaaaagggggaagatacccaggtaagagggcatgcatgctagctttccaatactttgatattacctgctttttctaagactgtatcaacctgtcgcccacccataacctatcttttcataacagagtccaactaaacctaaaaattaaaactggaacctagcagcttctacgcaatctaagaatactttgttccctctctcaaaatctttccctgcttttgaataattgacttttgaattcataaaaaccttcccttattaatcatcctattacttgcatcatagtaaaccctgatcaactcttaaaacattaaaagacattactatatttcttaatgaatacacaagacctttaagtacaaatgcttttatattcagcccctgtaaagccatcagatgtttgaaagtttttaaacacgaaccaaagggtttaattttaagaacttagctaggaatgggtgaaatcctacccaattaatagagttctgcaaattagtaacaaagtgtaaaatgaaaggaagggtcccttggagatgtgaaattcttctattgagagtcctgtcttctttattcaagaagtttgtagccattttcagaattcactcaagaaccaacttcttaatttagatatcagcgaacaagtcatggcaaaaaatacacaaagagaaacaccaccacatcgaaaaggatgaaaagccagaggtccaaccagtaggagtgtttgggaagcccatttgccccagactgaggcctcacatcgaagttctgcctccctccctcgctaaagcctcgccgctcccggagaccatctcgaccatcaacacccggtgcgtccacctccatctcgctcctgcagcttcgtaacaaccctagaaaccgaaaatgcttaagttcccggactttggtgttcgccgcaccggaaactgagcggagtccggccgcctgcgcagtgc

SEQ ID NO: 11123 - RNA, 1813 nt, Homo sapiens
  source 1..1813: mol_type = other RNA
ctgaatagctgggactacaggtgcatgccaacatgcccagctaatttttttgtatttttttgtattttttaatagagatagggtttcaccaggttggccaggctggtgtcacaactcttgacctcaagtgatctaccacccttggcctcccaaagtgctgggattataggcgtgagccactgtgcccggccaacattaatattttttattagctactacagcttagagtagctgctatgggagtgtggcctttttgattaaatactagctgatcaaccctagaatataaattcttgttttataacatttagatttaaataacaataagaatgtaagctccatgaaggcaagaatgcctttttgttttgttcactgctgtgtctaaaataatgcctggctcaaatatttgttgaatgagtaaatatgctgactttgctgaagtatttaagcaagttacagatattatacaagtaaatattttgggcacaagcacacttaatgaaacagtaaaaaaaaaataggtttgaaacacataatccttcgttataggaggctcaagagtttaaaaggaaaaaagggggaagatacccaggtaagagggcatgcatgctagctttccaatactttgatattacctgctttttctaagactgtatcaacctgtcgcccacccataacctatcttttcataacagagtccaactaaacctaaaaattaaaactggaacctagcagcttctacgcaatctaagaatactttgttccctctctcaaaatctttccctgcttttgaataattgacttttgaattcataaaaaccttcccttattaatcatcctattacttgcatcatagtaaaccctgatcaactcttaaaacattaaaagacattactatatttcttaatgaatacacaagacctttaagtacaaatgcttttatattcagcccctgtaaagccatcagatgtttgaaagtttttaaacacgaaccaaagggtttaattttaagaacttagctaggaatgggtgaaatcctacccaattaatagagttctgcaaattagtaacaaagtgtaaaatgaaaggaagggtcccttggagatgtgaaattcttctattgagagtcctgtcttctttattcaagaagtttgtagccattttcagaattcactcaagaaccaacttcttaatttagatatcagcgaacaagtcatggcaaaaaatacacaaagagaaacaccaccacatcgaaaaggatgaaaagccagaggtccaaccagtaggagtgtttgggaagcccatttgccccagactgaggcctcacatcgaagttctgcctccctccctcgctaaagcctcgccgctcccggagaccatctcgaccatcaacacccggtgcgtccacctccatctcgctcctgcagcttcgtaacaaccctagaaaccgaaaatgcttaagttcccggactttggtgttcgccgcaccggaaactgagcggagtccggccgcctgcgcagtgcgccgcgccccgggttccggaatgcactctgaacctactcttcccagcgcgcaggcgcctggctcggctttccgctgcctccgtgaccgcaattgtgaaaacttcacatttaacttgtctccaccttctatgtcatgttttcttcttggggagagggttattttctcaagatcaaggcagtgaatgaagtatttgtttccatagttttttgccttcctttggcacctattatttccctctacattctgtaatggtctcctattaatggggctatttattagactggtcat

SEQ ID NO: 11124 - RNA, 3815 nt, Homo sapiens
  source 1..3815: mol_type = other RNA
ctgaatagctgggactacaggtgcatgccaccacacccacctagagaaaattttttaaaaaatgaatagtctcaggaattcacggacaatgtcaaaagctctaacattcatgttatcaatgacacagaagtacaggacagtatggtacagaaaacaatacttgaagaaatcatagctgagaacttcccagatatctgaaacacaatcaagtggctctgtgaactctgataaggataaccgaaagaaatccatgtccatatacatcataattaaactgatgagaaccaaagacaaggagaaaatcttaaaaagcagctggggaaaaataaagcattacctgttgggaaacaatagttagaatgcctctggatttctgagaaaaaaccatggaggccagaaggcatagaacaattttttttttttttttgagatggagtcttgctctgttgcccaggctggagtgcaatgtcctgatcttggctcactgcaacctctgcctcccgggttcaagtaattctcctgtttcattctctaatctcagtagctgggattacaggcacttgccactacgccctgctttcgtatttttagcagagacaaggcttttgccatgttggccaggctggtctcgaacacttgacctcaagtgatctggccacctcggcctcccaaagtgttgggattacaggcatgagccaccacgcccggcctcaattgtatttctatatactaataatgagcaattggaaaaaaaatctacaatagccacccccccgccaagtgaaatatagtttgagacccattcatggatctcaaatccaaaaatgtgaaatgctcaaaatctaaaactttttgagagctgaaatgactatcaaaggaaatactcatttaagcattctggattttagagttgggatgctcaagtaatatttgcttcaggtaaagcaaatattaacctgaaaataatccaaaatatttctggtcccaagcatttctttttttcttttctttttctttttttttttttttctttttgagatggagtctcactcttgttgcccaggctggagtgcaatggtgcaagctcggctcactgcaacctccgcctcctgggttcaagcaattctcctgcctcagcctcccaagtaactgggattacaggcacccagctgttaaaagaaaaagcatttggcttctactggaatctggagccacagtttggtgtcaaacagagcagctgtgcttttgtttcaaatgctgtttgctgaaaacctctggatcagaagagctggtcttcagccaggtccttggcaccaagaggatgtgaacaatcctgaattccagggcctactgatggagtccactagttagtccctttgacacggcccccttatggatcccagtagtcagccggggtgcaggttttcatagtgattctaaacaaggctgcagtcactgtttagaagtgattgggggaagctggaactgtgctccttgtttcaggacctctagattgcacctagattaaacaagacggaagctctcaaaaggctctaagtctaggcctcctgtgaggtagggtctgaaaggacttaaaccatttttttttttttttttttttacacacagggtaactttttggaagagtactttgtaacaataaagtgctgtgcacagaaaggagaaatgccattatggggatgtgtgtgccgacctgggaccagcagggtgaaagagtctatcattcatgatgagagctgccatttgcgctaagcacacaccatgtgccaggcactatgccaagaaattgttgaatcttcacaataactctgtgagaaaagggctgtcattggacagatgaggacactgatgctcccaggggtccacatcacatgaagaggaggtgacagggctgggccttggtccgaagctccagccttccaagccaaggcctgtgagaggaaccgctgagacctgatgttaggcctgtttttctcatgtgccctggagaaggggactaacaccatcttttgccaaagtttggtgagggatggccaagagctctttgaaactttgccatgtacaatagcactcacaattttttttaaattttttatacagtggtatcggggtacagtggctcatcaacactttgggaggctgaggcgtgaggattgcttgaggccaggagtttgagaccagtctgggcgacatagtaaaatctcatctctataaaaaaagaaaaaaaatgaggcgggcatggtggcaaacatctgtagtcccagccacgcaggaggctaaggtaagaggatcacttgagcctgagaggttgtggctacagtgagccatgatcacactactgcactctaggatgggtgacagagcaggacagtttcaaaaaaagacaaaaaaaaatttacacagtggaatgctttctttaaaaactatcttatgcataagtacaatctagaaaaccagaactgggccacttatagtgaaggtggaagcagaggtggcctgggaccccccaggattcctggagcactgcctgaaggccatttatctagtagattggcactcactgtaagaagcgcaagaggtaccatgatgcttaaggctctggctctgggtgtgaaagaatgaggtggaattgtagcagattcattcctgggtcaatctgtttttggggagggctgcaggattccaggcctgccatgtgcaatgggtgctgccctctttcttctgggcaccatctgcctcaacctatcccctggccagtgtcactcacagggcagaaaatttatcttcaccatctcacaattagtttaatctctgactccaatgcaggggctcgtgggatggctcacagtggaatcatcaaacggacttccttctcatagatgtcagggatcattcccactggggaactgaccatgtgcacagtgttcttgccaaacaattggaactcatagtggatgagctgctcccaaaagccgctgttgggtcggatgatgggccggcatgacttggtccacgtgtgggcgtccagcagggacatggcgtggtacttcatgaggtaggcgaggcacagggcagctgagcggctcacaccagcagcacagtgcagcaaagtacggccctgcttcatctccacgctccactgagacattgatgaccatggtgatctggttgctagacagcatgagcttgttgttggcggccacaccattgctgatatacaggcttttggttatctgcgagaggccgctgactgagggctgccggaactgaactgggaaggcacacgagggtgctgtcatcaaggcggtgggtcagtggtcagcagtcagcgaagcacgaaggctgcgtctttctgctaggctgtgtccatggaaaactctctccttcaggcgggtgggcgggttcgctcaggaagtagccgcttggggaagccttaggcaaggttcttcgggagagagacccgtcatgatcccgcagcctcaatccccgctggcctaacgctttggtttccatagcaatgggctcgtcgcagaaaggaatagcctgtgccgggtcttcagagaaatcctggcctcggctccacgcccctgagcagccccaccctggctcaacctgttacccgccctgccggcaagccggggtcactgcagtccccgtggcgaagcagggtcagctcagctcaccgcaccccactccatccagccctgcccatctctacggcaacgggccgggtcgcaccagggctgcagccgagagacagtctcaccgcttccgtagccgcccgggctctgtgc

SEQ ID NO: 11125 - RNA, 3931 nt, Homo sapiens
  source 1..3931: mol_type = other RNA
ctgaatagctgggactacaggtgcatgccaccacacccacctagagaaaattttttaaaaaatgaatagtctcaggaattcacggacaatgtcaaaagctctaacattcatgttatcaatgacacagaagtacaggacagtatggtacagaaaacaatacttgaagaaatcatagctgagaacttcccagatatctgaaacacaatcaagtggctctgtgaactctgataaggataaccgaaagaaatccatgtccatatacatcataattaaactgatgagaaccaaagacaaggagaaaatcttaaaaagcagctggggaaaaataaagcattacctgttgggaaacaatagttagaatgcctctggatttctgagaaaaaaccatggaggccagaaggcatagaacaattttttttttttttttgagatggagtcttgctctgttgcccaggctggagtgcaatgtcctgatcttggctcactgcaacctctgcctcccgggttcaagtaattctcctgtttcattctctaatctcagtagctgggattacaggcacttgccactacgccctgctttcgtatttttagcagagacaaggcttttgccatgttggccaggctggtctcgaacacttgacctcaagtgatctggccacctcggcctcccaaagtgttgggattacaggcatgagccaccacgcccggcctcaattgtatttctatatactaataatgagcaattggaaaaaaaatctacaatagccacccccccgccaagtgaaatatagtttgagacccattcatggatctcaaatccaaaaatgtgaaatgctcaaaatctaaaactttttgagagctgaaatgactatcaaaggaaatactcatttaagcattctggattttagagttgggatgctcaagtaatatttgcttcaggtaaagcaaatattaacctgaaaataatccaaaatatttctggtcccaagcatttctttttttcttttctttttctttttttttttttttctttttgagatggagtctcactcttgttgcccaggctggagtgcaatggtgcaagctcggctcactgcaacctccgcctcctgggttcaagcaattctcctgcctcagcctcccaagtaactgggattacaggcacccagctgttaaaagaaaaagcatttggcttctactggaatctggagccacagtttggtgtcaaacagagcagctgtgcttttgtttcaaatgctgtttgctgaaaacctctggatcagaagagctggtcttcagccaggtccttggcaccaagaggatgtgaacaatcctgaattccagggcctactgatggagtccactagttagtccctttgacacggcccccttatggatcccagtagtcagccggggtgcaggttttcatagtgattctaaacaaggctgcagtcactgtttagaagtgattgggggaagctggaactgtgctccttgtttcaggacctctagattgcacctagattaaacaagacggaagctctcaaaaggctctaagtctaggcctcctgtgaggtagggtctgaaaggacttaaaccatttttttttttttttttttttacacacagggtaactttttggaagagtactttgtaacaataaagtgctgtgcacagaaaggagaaatgccattatggggatgtgtgtgccgacctgggaccagcagggtgaaagagtctatcattcatgatgagagctgccatttgcgctaagcacacaccatgtgccaggcactatgccaagaaattgttgaatcttcacaataactctgtgagaaaagggctgtcattggacagatgaggacactgatgctcccaggggtccacatcacatgaagaggaggtgacagggctgggccttggtccgaagctccagccttccaagccaaggcctgtgagaggaaccgctgagacctgatgttaggcctgtttttctcatgtgccctggagaaggggactaacaccatcttttgccaaagtttggtgagggatggccaagagctctttgaaactttgccatgtacaatagcactcacaattttttttaaattttttatacagtggtatcggggtacagtggctcatcaacactttgggaggctgaggcgtgaggattgcttgaggccaggagtttgagaccagtctgggcgacatagtaaaatctcatctctataaaaaaagaaaaaaaatgaggcgggcatggtggcaaacatctgtagtcccagccacgcaggaggctaaggtaagaggatcacttgagcctgagaggttgtggctacagtgagccatgatcacactactgcactctaggatgggtgacagagcaggacagtttcaaaaaaagacaaaaaaaaatttacacagtggaatgctttctttaaaaactatcttatgcataagtacaatctagaaaaccagaactgggccacttatagtgaaggtggaagcagaggtggcctgggaccccccaggattcctggagcactgcctgaaggccatttatctagtagattggcactcactgtaagaagcgcaagaggtaccatgatgcttaaggctctggctctgggtgtgaaagaatgaggtggaattgtagcagattcattcctgggtcaatctgtttttggggagggctgcaggattccaggcctgccatgtgcaatgggtgctgccctctttcttctgggcaccatctgcctcaacctatcccctggccagtgtcactcacagggcagaaaatttatcttcaccatctcacaattagtttaatctctgactccaatgcaggggctcgtgggatggctcacagtggaatcatcaaacggacttccttctcatagatgtcagggatcattcccactggggaactgaccatgtgcacagtgttcttgccaaacaattggaactcatagtggatgagctgctcccaaaagccgctgttgggtcggatgatgggccggcatgacttggtccacgtgtgggcgtccagcagggacatggcgtggtacttcatgaggtaggcgaggcacagggcagctgagcggctcacaccagcagcacagtgcagcaaagtacggccctgcttcatctccacgctgtggatatggtcagcaatagggtcaaagaagtcacagagacgtgagttaggggagtcagccacaggtacctgcatgtactggatatcctcatacaaggtgttcactacctccactgagacattgatgaccatggtgatctggttgctagacagcatgagcttgttgttggcggccacaccattgctgatatacaggcttttggttatctgcgagaggccgctgactgagggctgccggaactgaactgggaaggcacacgagggtgctgtcatcaaggcggtgggtcagtggtcagcagtcagcgaagcacgaaggctgcgtctttctgctaggctgtgtccatggaaaactctctccttcaggcgggtgggcgggttcgctcaggaagtagccgcttggggaagccttaggcaaggttcttcgggagagagacccgtcatgatcccgcagcctcaatccccgctggcctaacgctttggtttccatagcaatgggctcgtcgcagaaaggaatagcctgtgccgggtcttcagagaaatcctggcctcggctccacgcccctgagcagccccaccctggctcaacctgttacccgccctgccggcaagccggggtcactgcagtccccgtggcgaagcagggtcagctcagctcaccgcaccccactccatccagccctgcccatctctacggcaacgggccgggtcgcaccagggctgcagccgagagacagtctcaccgcttccgtagccgcccgggctctgtgcgcatgt

SEQ ID NO: 11126 - RNA, 4065 nt, Homo sapiens
  source 1..4065: mol_type = other RNA
ctgaatagctgggactacaggtgcatgccaccacacccacctagagaaaattttttaaaaaatgaatagtctcaggaattcacggacaatgtcaaaagctctaacattcatgttatcaatgacacagaagtacaggacagtatggtacagaaaacaatacttgaagaaatcatagctgagaacttcccagatatctgaaacacaatcaagtggctctgtgaactctgataaggataaccgaaagaaatccatgtccatatacatcataattaaactgatgagaaccaaagacaaggagaaaatcttaaaaagcagctggggaaaaataaagcattacctgttgggaaacaatagttagaatgcctctggatttctgagaaaaaaccatggaggccagaaggcatagaacaattttttttttttttttgagatggagtcttgctctgttgcccaggctggagtgcaatgtcctgatcttggctcactgcaacctctgcctcccgggttcaagtaattctcctgtttcattctctaatctcagtagctgggattacaggcacttgccactacgccctgctttcgtatttttagcagagacaaggcttttgccatgttggccaggctggtctcgaacacttgacctcaagtgatctggccacctcggcctcccaaagtgttgggattacaggcatgagccaccacgcccggcctcaattgtatttctatatactaataatgagcaattggaaaaaaaatctacaatagccacccccccgccaagtgaaatatagtttgagacccattcatggatctcaaatccaaaaatgtgaaatgctcaaaatctaaaactttttgagagctgaaatgactatcaaaggaaatactcatttaagcattctggattttagagttgggatgctcaagtaatatttgcttcaggtaaagcaaatattaacctgaaaataatccaaaatatttctggtcccaagcatttctttttttcttttctttttctttttttttttttttctttttgagatggagtctcactcttgttgcccaggctggagtgcaatggtgcaagctcggctcactgcaacctccgcctcctgggttcaagcaattctcctgcctcagcctcccaagtaactgggattacaggcacccagctgttaaaagaaaaagcatttggcttctactggaatctggagccacagtttggtgtcaaacagagcagctgtgcttttgtttcaaatgctgtttgctgaaaacctctggatcagaagagctggtcttcagccaggtccttggcaccaagaggatgtgaacaatcctgaattccagggcctactgatggagtccactagttagtccctttgacacggcccccttatggatcccagtagtcagccggggtgcaggttttcatagtgattctaaacaaggctgcagtcactgtttagaagtgattgggggaagctggaactgtgctccttgtttcaggacctctagattgcacctagattaaacaagacggaagctctcaaaaggctctaagtctaggcctcctgtgaggtagggtctgaaaggacttaaaccatttttttttttttttttttttacacacagggtaactttttggaagagtactttgtaacaataaagtgctgtgcacagaaaggagaaatgccattatggggatgtgtgtgccgacctgggaccagcagggtgaaagagtctatcattcatgatgagagctgccatttgcgctaagcacacaccatgtgccaggcactatgccaagaaattgttgaatcttcacaataactctgtgagaaaagggctgtcattggacagatgaggacactgatgctcccaggggtccacatcacatgaagaggaggtgacagggctgggccttggtccgaagctccagccttccaagccaaggcctgtgagaggaaccgctgagacctgatgttaggcctgtttttctcatgtgccctggagaaggggactaacaccatcttttgccaaagtttggtgagggatggccaagagctctttgaaactttgccatgtacaatagcactcacaattttttttaaattttttatacagtggtatcggggtacagtggctcatcaacactttgggaggctgaggcgtgaggattgcttgaggccaggagtttgagaccagtctgggcgacatagtaaaatctcatctctataaaaaaagaaaaaaaatgaggcgggcatggtggcaaacatctgtagtcccagccacgcaggaggctaaggtaagaggatcacttgagcctgagaggttgtggctacagtgagccatgatcacactactgcactctaggatgggtgacagagcaggacagtttcaaaaaaagacaaaaaaaaatttacacagtggaatgctttctttaaaaactatcttatgcataagtacaatctagaaaaccagaactgggccacttatagtgaaggtggaagcagaggtggcctgggaccccccaggattcctggagcactgcctgaaggccatttatctagtagattggcactcactgtaagaagcgcaagaggtaccatgatgcttaaggctctggctctgggtgtgaaagaatgaggtggaattgtagcagattcattcctgggtcaatctgtttttggggagggctgcaggattccaggcctgccatgtgcaatgggtgctgccctctttcttctgggcaccatctgcctcaacctatcccctggccagtgtcactcacagggcagaaaatttatcttcaccatctcacaattagtttaatctctgactccaatgcaggggctcgtgggatggctcacagtggaatcatcaaacggacttccttctcatagatgtcagggatcattcccactggggaactgaccatgtgcacagtgttcttgccaaacaattggaactcatagtggatgagctgctcccaaaagccgctgttgggtcggatgatgggccggcatgacttggtccacgtgtgggcgtccagcagggacatggcgtggtacttcatgaggtaggcgaggcacagggcagctgagcggctcacaccagcagcacagtgcagcaaagtacggccctgcttcatctccacgctgtggatatggtcagcaatagggtcaaagaagtcacagagacgtgagttaggggagtcagccacaggtacctgcatgtactggatatcctcatacaaggtgttcactacctccactgagacattgatgaccatggtgatctggttgctagacagcatgagcttgttgttggcggccacaccattgctgatatacaggcttttggttatctgcgagaggccgctgactgagggctgccggaactgaactgggaaggcacacgagggtgctgtcatcaaggcggtgggtcagtggtcagcagtcagcgaagcacgaaggctgcgtctttctgctaggctgtgtccatggaaaacttaaaaggatgttgtgaaattaaacgagataatccacgtaaagagttttctcagggcttggcatagagtaagccctctcaaaatgataactatttttctcgcttctgatagggaagttaaaatgcagggctctctctccttcaggcgggtgggcgggttcgctcaggaagtagccgcttggggaagccttaggcaaggttcttcgggagagagacccgtcatgatcccgcagcctcaatccccgctggcctaacgctttggtttccatagcaatgggctcgtcgcagaaaggaatagcctgtgccgggtcttcagagaaatcctggcctcggctccacgcccctgagcagccccaccctggctcaacctgttacccgccctgccggcaagccggggtcactgcagtccccgtggcgaagcagggtcagctcagctcaccgcaccccactccatccagccctgcccatctctacggcaacgggccgggtcgcaccagggctgcagccgagagacagtctcaccgcttccgtagccgcccgggctctgtgcgcatgtgc

SEQ ID NO: 11127 - RNA, 2370 nt, Homo sapiens
  source 1..2370: mol_type = other RNA
ctgaatagctgggactacaggtgcatgccaccacacccagctagaggcaatgattcttaaagtctccgctggctatctaggactcttattaaatatcctgttactttaaaaaggccatccaaatatattttcttgaaagaaacatttatttatgatctttattggtgaaataatttcaaacaaatccagaacaggttctcacactttgagcctttagtgcaaaaacattatgccatgcgggaaataaaatgcttatccagtggagcgctcccctgatgcattgaaatattaggatactcaagcagaagacgacttatgtgacagaaatctgctcataaatctgcttgaaaaagggcatgataaacctcatattaaggtttctcacaacataaatatgcttaagcaacttaattccaacttaatttcaaaacaccccaggaatcaactatccctttaaataaaaaaaataatcaatttatattcttcttaaaagaactccaacaatttaaaataagttccaattccatatatatatatatatatatatatatatatatatatatatatatatatacacacacacgcacacacacacatttataacttaggtgctcttttgcgctatatactttaattcatgcaaaagtgatagaggactggacttgaggctctacagaggcctttctgagaaagctgtgtagctccttactctggcgaagaacaagggggtgtacatcttgtcaatctcaaaagcactgactgcagtctcaccagttgatttgtaagtaatgtgacaagaatgatgtatccagatgagtttgttgaacctctggtgaccactggaacatagctgtagccccacatgaaaactctgatctgcttcttgtacagggacacgacgaaaatatctgtatttatagtcaagtggtttttcttcttttttcttagttattacagcaaatactttggtctgattgtctgtgtcttgtgacaagcgatagtgacccagtagaattgcatcagtcctggtattcctagttcttaaacgtggaacaatggactgaggctcttcaggggttgtcaacatcatcacatggccatcaggaaagaatcttatgtacctgtaatattccacttggtgccaggctctatagaaaccatcaagagactgttccccttgacgaatatatgtggttttactgatatacacgccatcaaaccgaacacgaggccgttctaaaaacatctctctccaggacgtgtacggaacaagtttaatacagcttctgccccaaactttcaagcaggccagacgccatatttcagggtctctggcacagatgtagaatcctctgcacaccagcgacaactgctccaatgatctgaggtccaagtcactagacaccacccatcggaagatgtacatcaggacctccattggcagcactgatatgtgaatctgactgctctcaagctcaggctgacacagtttaagcacagactcctgaaatgtgagttgctgctggaagtaggacaagagatctgccattttgctgtcatcatcattatcttcaatgtagctgtttccaacgccatcaccatctggagaccgggtataagtaatcttgaactctatatcaggtacaagttgcatagccctacgataaaacttgatggcttcatagagagctccattttgttcttcttctactgcttttaggaagagttctcgagccttttcttcttttgcctgttcttgttttcctttggtatctgccgatgttttctggagagagcctcttgctgctctgcaaggtcgattttctaaattgctagagcttacacctggagcaagttcaaacatccactgagctcggaacatctggagttgtgcctgcagatctgtttcagcaggactttcattttcttcatcatcatctgctctgacagtatcagaatgacaatcttcctcagcttctgccatgctggcggggcggcctgctgcgctcgaggggctctccgtgccccctctgcaccgccccccggaggaggggtgctgggtgtccgggtgtctactcctgcctgtctctgcagcggagcttagcagagttctcggtcggagaagcgcaccaggcagcggcaataactgcgggcccggcgtacggcagccatcttcgcggggcagggggccagatcggggcgcgctggggtggcggcggctgccggggactcggggagtggagggacgcccgttgccagccgaggcgggggattgtgcgagcaccggagcgtcagccctactggagaccccggacgccgccgcggagctgccccctcagctgcggaaacctgcgccgacgcgccgagcat

SEQ ID NO: 11128 - RNA, 2192 nt, Homo sapiens
  source 1..2192: mol_type = other RNA
ctgaatagctgggactacaggtgcatgccaccacacccagctagaggcaatgattcttaaagtctccgctggctatctaggactcttattaaatatcctgttactttaaaaaggccatccaaatatattttcttgaaagaaacatttatttatgatctttattggtgaaataatttcaaacaaatccagaacaggttctcacactttgagcctttagtgcaaaaacattatgccatgcgggaaataaaatgcttatccagtggagcgctcccctgatgcattgaaatattaggatactcaagcagaagacgacttatgtgacagaaatctgctcataaatctgcttgaaaaagggcatgataaacctcatattaaggtttctcacaacataaatatgcttaagcaacttaattccaacttaatttcaaaacaccccaggaatcaactatccctttaaataaaaaaaataatcaatttatattcttcttaaaagaactccaacaatttaaaataagttccaattccatatatatatatatatatatatatatatatatatatatatatatatatacacacacacgcacacacacacatttataacttaggtgctcttttgcgctatatactttaattcatgcaaaagtgatagaggactggacttgaggctctacagaggcctttctgagaaagctgtgtagctccttactctggcgaagaacaagggggtgtacatcttgtcaatctcaaaagcactgactgcagtctcaccagttgatttgtaagtaatgtgacaagaatgatgtatccagatgagtttgttgaacctctggtgaccactggaacatagctgtagccccacatgaaaactctgatctgcttcttgtacagggacacgacgaaaatatctgtatttatagtcaagtggtttttcttcttttttcttagttattacagcaaatactttggtctgattgtctgtgtcttgtgacaagcgatagtgacccagtagaattgcatcagtcctggtattcctagttcttaaacgtggaacaatggactgaggctcttcaggggttgtcaacatcatcacatggccatcaggaaagaatcttatgtacctgtaatattccacttggtgccaggctctatagaaaccatcaagagactgttccccttgacgaatatatgtggttttactgatatacacgccatcaaaccgaacacgaggccgttctaaaaacatctctctccaggacgtgtacggaacaagtttaatacagcttctgccccaaactttcaagcaggccagacgccatatttcagggtctctggcacagatgtagaatcctctgcacaccagcgacaactgctccaatgatctgaggtccaagtcactagacaccacccatcggaagatgtacatcaggacctccattggcagcactgatatgtgaatctgactgctctcaagctcaggctgacacagtttaagcacagactcctgaaatgtgagttgctgctggaagtaggacaagagatctgccattttgctgtcatcatcattatcttcaatgtagctgtttccaacgccatcaccatctggagaccgggtataagtaatcttgaactctatatcaggtacaagttgcatagccctacgataaaacttgatggcttcatagagagctccattttgttcttcttctactgcttttaggaagagttctcgagccttttcttcttttgcctgttcttgttttcctttggtatctgccgatgttttctggagagagcctcttgctgctctgcaaggtcgattttctaaattgctagagcttacacctggagcaagttcaaacatccactgagctcggaacatctggagttgtgcctgcagatctgtttcagcaggactttcattttcttcatcatcatctgctctgacagtatcagaatgacaatcttcctcagcttctgcctcaaaaatttttacaacccaaatttaggggtgggcccttaaagcaagccgccctgagaagcatcgaactggacgcttgggacagtcgctacaaagtcctcggagcctctggctagagtcccgcgccaggaatgcaggaaaacagtgaaatttctcaacagtcacagttgttataacgactaaagtttttgagagcacagacagactggag

SEQ ID NO: 11129 - RNA, 2065 nt, Homo sapiens
  source 1..2065: mol_type = other RNA
ctgaatagctgggactacaggtgcatgccaccacacccagctagaggcaatgattcttaaagtctccgctggctatctaggactcttattaaatatcctgttactttaaaaaggccatccaaatatattttcttgaaagaaacatttatttatgatctttattggtgaaataatttcaaacaaatccagaacaggttctcacactttgagcctttagtgcaaaaacattatgccatgcgggaaataaaatgcttatccagtggagcgctcccctgatgcattgaaatattaggatactcaagcagaagacgacttatgtgacagaaatctgctcataaatctgcttgaaaaagggcatgataaacctcatattaaggtttctcacaacataaatatgcttaagcaacttaattccaacttaatttcaaaacaccccaggaatcaactatccctttaaataaaaaaaataatcaatttatattcttcttaaaagaactccaacaatttaaaataagttccaattccatatatatatatatatatatatatatatatatatatatatatatatatacacacacacgcacacacacacatttataacttaggtgctcttttgcgctatatactttaattcatgcaaaagtgatagaggactggacttgaggctctacagaggcctttctgagaaagctgtgtagctccttactctggcgaagaacaagggggtgtacatcttgtcaatctcaaaagcactgactgcagtctcaccagttgatttgtaagtaatgtgacaagaatgatgtatccagatgagtttgttgaacctctggtgaccactggaacatagctgtagccccacatgaaaactctgatctgcttcttgtacagggacacgacgaaaatatctgtatttatagtcaagtggtttttcttcttttttcttagttattacagcaaatactttggtctgattgtctgtgtcttgtgacaagcgatagtgacccagtagaattgcatcagtcctggtattcctagttcttaaacgtggaacaatggactgaggctcttcaggggttgtcaacatcatcacatggccatcaggaaagaatcttatgtacctgtaatattccacttggtgccaggctctatagaaaccatcaagagactgttccccttgacgaatatatgtggttttactgatatacacgccatcaaaccgaacacgaggccgttctaaaaacatctctctccaggacgtgtacggaacaagtttaatacagcttctgccccaaactttcaagcaggccagacgccatatttcagggtctctggcacagatgtagaatcctctgcacaccagcgacaactgctccaatgatctgaggtccaagtcactagacaccacccatcggaagatgtacatcaggacctccattggcagcactgatatgtgaatctgactgctctcaagctcaggctgacacagtttaagcacagactcctgaaatgtgagttgctgctggaagtaggacaagagatctgccattttgctgtcatcatcattatcttcaatgtagctgtttccaacgccatcaccatctggagaccgggtataagtaatcttgaactctatatcaggtacaagttgcatagccctacgataaaacttgatggcttcatagagagctccattttgttcttcttctactgcttttaggaagagttctcgagccttttcttcttttgcctgttcttgttttcctttggtatctgccgatgttttctggagagagcctcttgctgctctgcaaggtcgattttctaaattgctagagcttacacctggagcaagttcaaacatccactgagctcggaacatctggagttgtgcctgcagatctgtttcagcaggactttcattttcttcatcatcatctgctctgacagtatcagaatgacaatcttcctcagcttctgcctgaggggggaaaacccaaataatgtcaggcatataaacacaccagttgccctctgcaatctacatttctcattcagccacttt

SEQ ID NO: 11130 - RNA, 829 nt, Homo sapiens
  source 1..829: mol_type = other RNA
ctgaatagctgggactacaggtgcatgccaccacacccagctagtttttgtatttagtagagaaagggtttcgccatgttgcccaggctggtcttaaactgctgagctcaagcaatccacctgccttggcctcccaaactgttgggattacaggagtgagccactgtgcatggccctggatggctttttgttgttgttgctgttttttctgattccattttccctctggtcttctacaagtgtctgagaacataggctggagaagcaagctggcacatgtctgttggttccatttaggcatgtggattgattgtcctctcatctggccatctccaaaatggctgccatgtgtcacatgttatggcctttctacacagtcatgatttatgacgtcagagatgaactggaatataggctcctaggaaatattctcccacaggaaagtacaggcttgtgtgagaagccaccacggcagacaatcctgagtagcgggcagaaaccggcttgcgtctctgaatacacttgttcctctgccttcccaactcctatgcatacttttgaggccattctcgggtagcccctctcctctccgaggcctgtccttatgacgcctgcccgctgtggcactccggttacccggaggagagttgctactctcgagttcaccgaggcggaaagcccctctgactccaaagcagggctcagcgcgacgtcccagaggccgcttctagtggcaggtgcccctcctcacagggccctcgcagccccgccggcccccgcccggctccttctcagcatgatacaaccgcgtcggccctggacagcgcat

SEQ ID NO: 11131 - RNA, 4099 nt, Homo sapiens
  source 1..4099: mol_type = other RNA
ctgaatagctgggactacaggtgcatgccaccacacccggctaattttttgtagtttagtagagacggggtttcaccgtgttgcctaggctggtctcgaactcctgagctcaggcaattcacctgcctcggcctcccaaagtgctaggattacaggcgtgtgccactgtgcccggctggttcaaacttttcatataacccttaggaaattggatgtgacagggagaaaagataggaccttttcagcatttcttaatatgcagaattgccaaatattccaaagatggtctagtgacataaaagtatattacaagtttgtttgagaacatctatatttaaatctaacctttaaacaattttaaattgatatttgttttaaatatgaattgactattgcccctttatcttagctatggtttggggaaacaagcatttttttatttccaaagaaatgttagaatttctatgctgaactgcattttaaaataaaatataatatttagctttaggtattttaattactacaaaggggagagctttgcatctaagcaatacttttcatcaatagatctccagttttctataggcagacggactccctctgtttgataaagaaggaaacaggcacagagaagttaagaccctcccagtgaagactaagccaggctctccatctcccatctgggagaagctgcttcatcctagagggtggtctcactgtcagtttctcttcggtatttatccatgtctgtgaagtcatagtctgactccatctctatcttcacctgtggcaccatgaacactgggttccgtgagtagctgaaagcaggtgaagctggacaggatattttgaagtgcaaggtgatgcttcggtcaagttctgtgtcactgaaggaagaatcagagtgagtaactccaactggaagatctttttctggcaatgcagtggataccgttttggggatctgattggacactttccatgggaatctttataaccgagggaggagggaactggggctcctcatcacagtcctcgtgggcccctttttttctcttcctcttcttgtctgtctcctttttttccttctctgggaggatgttgtcaatccaggccaggtcgtgctgggaaaagatgaaatccagaagccttcgaacgatgatgaggcccaggatcatgaccgggaagatgatggcagccaccgtggatttgaggatccagagcaccgccaggcagaggatctgcaccagggtgaagaggtggatccggcgcagcggcacgtgccgcaggaaggcatggtccggctggtgcttggctggcatcaggaagagcttgcagcgttcccagaactggatgccattcagggaggccacgcccatgtagaggaagactccgtacagcaccggcagggggatacactttaggatgggagccaggaagacagagattcccgtcaggatgaagacgatgatgccggttactctctgttccctgactcccagaaactggggctgctccccaggggcactggtctctgtctccatcttgaggctgtcgatgtgggcgatggagatgaccgtggcagccacgtaccaggggagccccataaaggagcacaaagccatgaggatgcccacccagaacaggtccagatggtagccggcagccttcttcagtttgttctccttccggttgacaatgacggcagtgatctgctggtccatgaagatcaggatggtcaccagcagggcgggcaggatgcttgctgggtatacccaccacgggttcttcccaaagggggccacgaaccagcctcggtcaggccgcgttggcttgatgacactgggcacatgcagcttgggagtttctaggccaaaacaggcatcgattccacagaacatcaggatggagaaaacaatggaaaagtcagccaccagggcccggaccttggtaggaaaatagcggctgaatttgaacttcttcagggtcagggtcatggagtatgtcccaaagaaaaggatgaaggacatgagcgccaggtctgggataaacttgcaggaattcccaagcaggcgcccgccgtagctcagacactccttcttgctcagcagggaccagtccaacgctgtgaggttaaggaggttgtacagagaagcgttggtgtctggtgccaatggggctgaagcattgaacacggttgtattcactgtgtcaggggcgacacactcgcacttgtaggtagtgatgaagtttggcttgaagtccatattgatagggtagtacttgaaggcaccgatcatcttcttgatggcatcgtagatgaagatgaagctgataagggtggagaagccctcctcggtgaagcgggtgatatatttgatgataaagctggcatctgtggccactaggataaggcactggacagctgagtgtaggccaatccagaggcggaactccatgtagtccaggccattgcctttgctgaagtcgaagaggagcttctcaaagatgaggatgggccccgtgctgctgagaatgatgagaggctgtcccgagaagaggcagaacaaggagccagccatggcagtgcccaggaagctctccatcactccctgataattgtcggtggcatcccccagaagcccaccaaaggtgatcgcgttggtgatacagccgaggtagatgaataggatggcagagatggactgaatgtggaagccatcatagaagtcacttgggaaccagggcaacttcctcttgatatccagacacaggccaccgaagaaccttcctgtccagataagttcctccccgatttcatgcatggctggcatctctccatcatccccgctgcttgttccgccggccccgccactgccagccccgccgccactgccaccaccaccaccacctccattgcctcctccaggagctccgccgcctcctcccacagagccattcatctggcccagctctgctagggagaacacagatttcctcttgtcagcagagggcaccttcttggggggctcaatccggatatttgggtcccattctccaggaggaaggacgatgacctcatccagaaattcatcaattcctgcgatcagatcttcccgattgcgggctttgtaggccacgtcactgaagagatcatctaccatgagggttgcaatggcacggccaatttcattgtaggattttgctctcccagaaggtcccagtagtataaacagaaatctggtggggacaggcacctcggtcactcctcccagcatggccgactggatgaggcgcacgaacgcgatgaatggctggtctaggaagtccacctcgcccacgagcacgttggacgcttctgagtccttggggatcttcttcatgaatttgtttttccgctggtctgtgtttggggtgagagaaatgtcattcatgcttctgctctgggcatgacacagacgtccgtaatttgcactctgccgcatccgcaggtcttccgtggagtggtgtagactcgggccagcaccagggctccgggcaggactgcgatttgtggtggagactgacttcccaatgtcagctaaggagcggtggatgggcttcttggtttggtggcggtgcctcctcaggaggacgtaactgaccctctcccggagctctggccgcaggagaccatcctcaatctgcttctcaatgacatcatctatgatctgtggtaaggagccactgtccaaatccagcagcaccgtccccgtctgcaggcaggtacggagctcgaagaggctgtgcagggatagtgtggacacgtggggcttgctccagcgttcgccgccttcctctaccttttcttcaaactttatccacctggctgactccttccactccatctggtctccgtcatgctgcagagtatccatctctgtaaagagggtggggttgggagcctcatcttcctcccccaggatgtcctggagctgctcagcagctggggaccctgctccctggaacagctgagcgctggggtccctggctgtcgatgctgcctctggccccagcctgcttccgctgctgcctccctggctgctacttccacaggtcc

SEQ ID NO: 11132 - RNA, 4672 nt, Homo sapiens
  source 1..4672: mol_type = other RNA
ctgaatagctgggactacaggtgcatgccaccacacccggctaattttttgtagtttagtagagacggggtttcaccgtgttgcctaggctggtctcgaactcctgagctcaggcaattcacctgcctcggcctcccaaagtgctaggattacaggcgtgtgccactgtgcccggctggttcaaacttttcatataacccttaggaaattggatgtgacagggagaaaagataggaccttttcagcatttcttaatatgcagaattgccaaatattccaaagatggtctagtgacataaaagtatattacaagtttgtttgagaacatctatatttaaatctaacctttaaacaattttaaattgatatttgttttaaatatgaattgactattgcccctttatcttagctatggtttggggaaacaagcatttttttatttccaaagaaatgttagaatttctatgctgaactgcattttaaaataaaatataatatttagctttaggtattttaattactacaaaggggagagctttgcatctaagcaatacttttcatcaatagatctccagttttctataggcagacggactccctctgtttgataaagaaggaaacaggcacagagaagttaagaccctcccagtgaagactaagccaggctctccatctcccatctgggagaagctgcttcatcctagagggtggtctcactgtcagtttctcttcggtatttatccatgtctgtgaagtcatagtctgactccatctctatcttcacctgtggcaccatgaacactgggttccgtgagtagctgaaagcaggtgaagctggacaggatattttgaagtgcaaggtgatgcttcggtcaagttctgtgtcactgaaggaagaatcagagtgagtaactccaactggaagatctttttctggcaatgcagtggataccgttttggggatctgattggacactttccatgggaatctttataaccgagggaggagggaactggggctcctcatcacagtcctcgtgggcccctttttttctcttcctcttcttgtctgtctcctttttttccttctctgggaggatgttgtcaatccaggccaggtcgtgctgggaaaagatgaaatccagaagccttcgaacgatgatgaggcccaggatcatgaccgggaagatgatggcagccaccgtggatttgaggatccagagcaccgccaggcagaggatctgcaccagggtgaagaggtggatccggcgcagcggcacgtgccgcaggaaggcatggtccggctggtgcttggctggcatcaggaagagcttgcagcgttcccagaactggatgccattcagggaggccacgcccatgtagaggaagactccgtacagcaccggcagggggatacactttaggatgggagccaggaagacagagattcccgtcaggatgaagacgatgatgccggttactctctgttccctgactcccagaaactggggctgctccccaggggcactggtctctgtctccatcttgaggctgtcgatgtgggcgatggagatgaccgtggcagccacgtaccaggggagccccataaaggagcacaaagccatgaggatgcccacccagaacaggtccagatggtagccggcagccttcttcagtttgttctccttccggttgacaatgacggcagtgatctgctggtccatgaagatcaggatggtcaccagcagggcgggcaggatgcttgctgggtatacccaccacgggttcttcccaaagggggccacgaaccagcctcggtcaggccgcgttggcttgatgacactgggcacatgcagcttgggagtttctaggccaaaacaggcatcgattccacagaacatcaggatggagaaaacaatggaaaagtcagccaccagggcccggaccttggtaggaaaatagcggctgaatttgaacttcttcagggtcagggtcatggagtatgtcccaaagaaaaggatgaaggacatgagcgccaggtctgggataaacttgcaggaattcccaagcaggcgcccgccgtagctcagacactccttcttgctcagcagggaccagtccaacgctgtgaggttaaggaggttgtacagagaagcgttggtgtctggtgccaatggggctgaagcattgaacacggttgtattcactgtgtcaggggcgacacactcgcacttgtaggtagtgatgaagtttggcttgaagtccatattgatagggtagtacttgaaggcaccgatcatcttcttgatggcatcgtagatgaagatgaagctgataagggtggagaagccctcctcggtgaagcgggtgatatatttgatgataaagctggcatctgtggccactaggataaggcactggacagctgagtgtaggccaatccagaggcggaactccatgtagtccaggccattgcctttgctgaagtcgaagaggagcttctcaaagatgaggatgggccccgtgctgctgagaatgatgagaggctgtcccgagaagaggcagaacaaggagccagccatggcagtgcccaggaagctctccatcactccctgataattgtcggtggcatcccccagaagcccaccaaaggtgatcgcgttggtgatacagccgaggtagatgaataggatggcagagatggactgaatgtggaagccatcatagaagtcacttgggaaccagggcaacttcctcttgatatccagacacaggccaccgaagaaccttcctgtccagataagttcctccccgatttcatgcatggctggcatctctccatcatccccgctgcttgttccgccggccccgccactgccagccccgccgccactgccaccaccaccaccacctccattgcctcctccaggagctccgccgcctcctcccacagagccattcatctggcccagctctgctagggagaacacagatttcctcttgtcagcagagggcaccttcttggggggctcaatccggatatttgggtcccattctccaggaggaaggacgatgacctcatccagaaattcatcaattcctgcgatcagatcttcccgattgcgggctttgtaggccacgtcactgaagagatcatctaccatgagggttgcaatggcacggccaatttcattgtaggattttgctctcccagaaggtcccagtagtataaacagaaatctggtggggacaggcacctcggtcactcctcccagcatggccgactggatgaggcgcacgaacgcgatgaatggctggtctaggaagtccacctcgcccacgagcacgttggacgcttctgagtccttggggatcttcttcatgaatttgtttttccgctggtctgtgtttggggtgagagaaatgtcattcatgcttctgctctgggcatgacacagacgtccgtaatttgcactctgccgcatccgcaggtcttccgtggagtggtgtagactcgggccagcaccagggctccgggcaggactgcgatttgtggtggagactgacttcccaatgtcagctaaggagcggtggatgggcttcttggtttggtggcggtgcctcctcaggaggacgtaactgaccctctcccggagctctggccgcaggagaccatcctcaatctgcttctcaatgacatcatctatgatctgtggtaaggagccactgtccaaatccagcagcaccgtccccgtctgcaggcaggtacggagctcgaagaggctgtgcagggatagtgtggacacgtggggcttgctccagcgttcgccgccttcctctaccttttcttcaaactttatccacctggctgactccttccactccatctggtctccgtcatgctgcagagtatccatctctgtaaagagggtggggttgggagcctcatcttcctcccccaggatgtcctggagctgctcagcagctggggaccgagtcctgctgataagatccatgctgctgtcctggctgcttgccccactccctgggccagtcagttcctgctgtggctggtctggccgcaggccccagtggactttttgcaggcctgaaagatgtcccttctggtcagtttttctttgagggtaagtgggtactggaagcccaatgtggataggagggcattctttctgatccggaaatctcctcctgtggttagtgtggtccagctttcctaccccagccttctcctccttcaccttcatgactttgtgttcttagctctggaaaccaggatccaaatcccagggaggccagaaccacttgctctgttccacagtatgtgcaatttttggcttccagattgtttgtgccaagctttggcaggtggtacaatattggctgccccagattcttgtctgctttagctgtttctgaaccatgtccagggttgagaagggaacatactgtgatggtgtcagcactcttttggtagcagcaactctttatctggaaggttatcttacactcccacctgggtggtcttcagggtactcctggaaacatccatcagctcatgagctcacagctgaattccaaatcctgggatgccccagtgcagtggcctgtggctcctgggccctgactccaattcctttagggtggaccttgc

SEQ ID NO: 11133 - RNA, 7042 nt, Homo sapiens
  source 1..7042: mol_type = other RNA
ctgaatagctgggactacaggtgcatgccaccacacctggctaatttttgtatttttagtagacatggtgttttattgtgctgcccaggctggtctcaaactcctgacctcaagtgatctgcctgcctcagccttccaaaatgctgagattacaggcatgagccacaatgcccagccaagaatctaataatttttggatcttgaaaattgtatttcttattagaaaaagtaaagaatcacaggcttacatcctatgatcacagatctaagtgttctggttgaaagaggaagaagaggcaacatacaaactacacttctgtggacaccaagtgtagtgtggcaggaaaacataaagtttgcatgtataaaaccttaaaagttgaatgcctacaatgtacttgtctgtggcaggtatgagagatcgaaaccttacaatgtcaatgggatcagacaagggctctattttgatcctggaaagcatcaccagctgtatacattgtattctatgcattctattttaaacccctggagcagctcagtggctcgctggctgaatactgagacactgacattactgcaggctaggatttccccctataggacagccacttgtgatacttaccccatcaaagttttcctccatcttactgtgacagaacctacatgagattcattcgggaaattctcaacaagaggactctatcctataagtcgtccccaatccccagatctccaatggattattcttgtaaacagcacttttaccttccgatcgctctaccacagaggccaaaaagggttttcccctaacatccaaatacctattcagataccagccctgctccttctcttaaaatctgtcttctcacctgggcgtggtggctaatgcctgtaatcccagcactttgggatgctgaggtcggtgatcacttgacatcaggagttcgagaccagcctgggcaacatggcaaaaccccatctctactaaaaatacaaaaattagctgggcatggtggcacgtgcctgtaatcccagctacttgggaggctgaggcaagagaatcgcttgaacccaggagcgggaggttgcagtgacctgagatcacgccactgcactccagcctgggcgaaagagtgagattgtgtctcaaaaaaataaaaatgtgtcttccacttcttaaaccccaaagctgttttgttgttgttgtcatttaaaacagacacagactatgcttccctcctgatttattaagaccgacatatttaatttgcatttcttgagggaatagcacctggaaaccagggagaaagaagctgaagcatgcaggtcatgaattattcaatttggtgtcaataatttgtcagaaaaattaaaaaaaatcaatagataaccgtattgtagttcaactgattataatatagaagcaacggataatgaacaccctttcctcaaagtcatttattctcaacctttggaaatgattacgtttttacctccagtgaatcccttcatcacagagaataacagggtaccagcccaagccaacagtgccccataccagagaactcagggaaacaaagaccctaaaggttatgtacaatgagagaatcagactgtgaggctccagctctcttctgtatccctgctcactttacctcagtgcacaccatatcccttcttcctccattgtgaaatgtgcatacacgtgtttgtctgtgaatatataaatatctctatttacacatatatacatatataaaaatgtgcaatacaaagacataagcaaggagtttttcctaataactatttaatcagagactgattggagaaaaaacaagttcttcccctcaaattttccttctaacttgagaaccaattcctggaccaattcctgctcaaagaaaacatttaagaagcacctgtcggctgggagtgctagctcacacctgtaatcccagcactttgggaggccgaggcgggtggtcacttgaggtcaggagtttgaaaacagcctgaccaacatggtgaaccacttctcatagagacacattattaacttggtgaaacttaattgggatgaggagcactctgtatacatgtatcatttctgtttttcctcattgtgatggttaatcttatgtgtcaacttgactaggccacatgatgcccagatatttggtcatacagtattctgggtgtgtctgtgaaggtgtttttggaagagactaacatttcagtcagtagactgaatacagcacatggccctccctaatgtaagtggccctcatccaatcagttgaaggtctgaatagaacaagtaagggagaagtcctcctgcctgactgcttgaactaagacctcagtcttttcctgcctctgaactggaacagaaacatcagctcttctagggtatccaagctggccttcagactggaactacaccatcagctctcctggatctctagctggcccactgcagatcttgggatttctcaaactccattattgtgtgaaccaattccttataataaatctcaggctgggcatggtggctcccgtctgtaatcccagcactttgggaggccacgactggcagatcacctgaggtctagagttcaagaccagcctggccaacaaggtaaaaccttgtctctactaaacatataaaaaattagctgggcatggtggcaggtgcctgtaatcccagctgcttgggaggctaaggcagaagaatcgctggaacccaggaggtggaggttgcagtgagctgagattgcaccactgcactccagcctaggcgacagagcaagcctccatctcaaaaaataaataaataaataaataaataaataaataataataataataataataaatccctgaagaatcctaactcctcaacataaattaacctggacatctgaggtgcctgccattataagaagaaacacaacagatccattaagtgggacaggtctgggaaacagtaaaatgagtctcacatcctctatccaccagagcaaaaaaagtgaagaaaacttcatgtaactttgtctgatgctgtttgctatactgtgtataaaaaggcagacccctatccagtactttgtttccaccctttttaaaggtactcagatcctttctagttctctaggcattggttctctatctgtacgtaaaactacaactgcctgtcctggcatctccagacactgacaagcaaatatgtccaggctgtcatgatttttctgagacaactgatattgtgtacttgaaaactgcaatgtgtcccaagttcaacatagccttcctccatctaagtagtggccaaatattcataatacacctctaatttccttccatcctcctccccaattcaaaaccagtgtgtattctcaagctacatttcaggggcaacgcacagtaagtagatctcattccccaaataaacaatcactacagaggtgtaatatgggaggtatatgaaaaaacatattttattccctctgggcccaaatgaatcatactttctggtcacaacttttagaggcaggctattatttcagcaggccactctctcactttttctgttccctctctgactccttcatcctttaccaaagtacagagaaacgttatctctagcccccttccgtcacccacaaatcagcgtatgatagtcaacaaaaactgaggaaagacttctagccaagaaaaagacccattaaagagtggtgtttttgttctgatcattctaaactgatcattctgatcattgttgtgtgacaatacaaatggtgcccctctgtacctttttttggtacaccaacagttgttctatgtccccatcatttccttttgagaccttgaagtttcaacaacattcttgaccttcttaatttatccaatgttaaacacttgaatgctacaaagagcatgtgcatgggacactactaggctgaaaaaataaggcctacctcttccaggccaagctgttttggacatgatcacactgatcagtttgagtccaagtatagccagaaccaaggagaaaaggaaagtttcagagatgaaaaataggcttaaaaattaaaatgtgacaatgtaaaatcttaactcctgaagaccaatgaattaccaaaaacagtgaactggctgcagacacttactgtctctatttctgtgaggcaaattattttaagattactaggaaaaaagacagtaaacaatgagttgagcactttgagaggttgaggcaggcagatcacttgagcccaggagtttgagaccagcctgggcaacacggcaaaaccctatctctacaaaaatacaaaaattacccaggcatggtggcacacgcctgtagtcccagccacttggtaggctgaggtgggaggatcacttgagcctgggaggtcgaggctgtggtgagctgagatcgtgccactgcactccagcctaggcgacagaaacaaacaaaaaaagcagtgagttggggattttttttttttttttgagatggagtttcgctcttgttgcccagactggagtgcattggtatgatccggctcaccgcaacctccacctcctgggttcaagcgattctcccacctcagcctcatgagtagctgggattacaggcatgcaccaccacgcccagctaattttatatttttagtagagacaaggttttaccttgttggccaggctggtcttgatctcttgaccttgtgatccgcctgcctcggcctcccaaagtgctgggattacaggcgtgagccaccgcgcccagcggtaatcattttttaaaatctcagaagcaaaggtctcaaacatctgtctttctgtgcctgtatgctgcccaactcattcccaaaaaggaatgggaatcagattcctatcaacataaggctcccaatatatgttatgtaggtttcttgggaaactgcatcaactgaagtagtctttaaaaattaaaataagaggccaggcgcagtggctcacgcctgtaatcccagcactttgggaggctgaggcaggcggagcacaaggtcaggagattgagaccatcctggctaacacggtgaaaccccatctctactaaatatacaaaaaattagctgggcatggtaacaaatgcctgtggtcccagctactccggaggctgaggtaggagaatcgcttgaactcaggaggcagagtttgcaatgagccaagatcgtgccactgcacttcagcctaggcgacagagcgagactccatctcaaaaaaaaaaaacaaaaaaaattaaaataagaaaaccaaagcacacaatgataaaccacttttctcttcttgctgtaatttttctttgatttgctctctggggatcaagacaaaacaaaatcattagtcttagatacctgaatttgacctcgcctcatagctaatgtgatcaagagtagttttttttttttttaaatacaattaagacaaaaggactttatatcagcaggactttagggctgtggttccactgtttttatagtaaaatacactaatggtggggtagaggttggagaaggaggtggaaacatccgttacaaggcaacatgacagacagcaggaccctaactagactttaaggaattaattctattcagacggggggagccctacataattaagtttcacacttataaaattatcactctgaattcagggataagaggcatttggttgtagatacaattccatctgtagatactaactttaaatttaaagaagaaaaacattcattgcatttatattatgtgttgagtttcttacatattcctaaatccatctactaattttttgttttgatacaatttacagctatggtaagatgattaccacagccctgattcaggtgtggtctttagcttcagaaagtccatcggtcatgtagctgactgtcattgctaaatctgttgcttgcagaggcctcagtgctctggctttgccgagtagagtcctcaccatttaagctcttcctacatacaggacatgtgtcatgcagttctagccacggcacaatacaactgctgtgaaagaagtgattgcaaggtaactgccggacttcctcttcaactgtgtaatcttctttgcatactggacactctaaacccatatcaacttgttcctgagttactgtcactgttggaagagatgtgatcttttccttgtcagctgggggagggcctgtgttttccagttgtcctaaaagctgggttacaatggcatcaagccctgtctgaccccaggcatagtccccagggttggagtgcagcatcccgctccaggaaaaagggtgtggagatccaggaatggcagaatttgcaaagaatcctgcaaagatgtgttgtagtattccttcaatagctggagatctgtcaggacgagaacttcctcgagatctgtatctccgacccaatggcaaccgtggaggtcttgctccccagaagtcagtgtgagtctggtgacccctttcattggctctattatcttggtccagtggactgctacttagaaagggtctaaaatcttgaaaaaacatcgtgtgatccaaatggccccaaagctctgcaaaatgtgttgttgtggtattgtctatccgactgccgccaccacctaaaaaactggaatcatctgtcacttcttcaataaagcctgattcacatctgggacatatatattccggtagtttggggctgacctcgcccttgcaaaagtggcagaaaaaccggtgggcggctacagcggcgcccgagtccgccccggccgccgaagcctccgccatttttgccctccgccgcggccgtccgagagggcagccggcccgtccctcgccaggccgctacctcccgagctgcagtcgtcgccgccgccgccgcctcggtgcggcccaccgcttcagagcccgcgtcggtcacgtgagttggccaggcccagaaacgcggcggcgccaacagctaccctgcggcccgcctcccagcaccaaagaggcgcaggaaggagagac

SEQ ID NO: 11134 - RNA, 3726 nt, Homo sapiens
  source 1..3726: mol_type = other RNA
ctgaatagctgggactacaggtgcatgccaccacacctggctaatttttgtatttttagtggagatggggtttcaccatgttagtcaggctggtcttgaactcctgacctcaagttatccacccacctcagcctcccaaaaatctgggattgcaggcgtgagccaccgcatccagcctaatgttttaatggcagacttgaataggcagaaaaaaaatccttaacgttaaagagagatcatttaaaattattgaggctaaggtgccaatagaaaaatgaatgaagaaaagtaaacagagactgaaagactatgggatactaccaaatgaaccaatatactcattatgaagttttaggagaagagagaaacaaagaacagagaacttacagtagtcctcttttatcaattgggtatgttccaacatcccaaatatagtatcaaaccctatatgtactacttacaaatttctttttcttccatcacaatttcatggatagatttacttttactgtagatcttagaaacctcgcataatttttttccttccttgtgtcaagaattttcaactttttacttaaaggaagcactccatgaacattttttttttggcatacccaaatttccagcattacctatattacactttggggactttgttaagtaaactaagagttgcttgaacaaaagcactgtgataccatgacagtcaatctgataactgagatggctactaaatgactaacaggcaggtagtatatacagtgtagatatcctagacagagggatgattcatgtcctaggtagaacagagcaggatagcacaagatttcatcatactgctcagtatggcatgtgatttaaacttataaattgcttatttctggaattttcatttaatattttcaaactgctgttgaccattggcaatggaaactgtggaaagtgaaactgtgggtgatggtaaactactgtgtttggagaaataatgaccccaaactgcccaaatttgagaaaagacatgaatctacaaatacaagaagctcaacaaactccaagtatgataatccaaagagatccaactaaaatatagtcaactgtgagaaatcaaagacaaaggaaatcttgaaaacagaaatggaaaaatagctatacaatgtgtcctcaataacactatcagcagatttctcagcaaaaaccttgcaaataaaaaagtagtgagataatatatttaaaatgctgaaagaaaaaaaaagttgtgactaagaattctatatccagcaatactgtccttcaaaagcaaagaattaaaacttcccagatttaaaaaaatgctgaggaaattcattactactagacctgttctgtaaggaatgtgaaagagaatcccttaagttaaaatgaatggatgctaggccatataaaattttctagcgaaggtaaaaatatgggcaaatgtaaaaactttcattattataattttggtttttaactcaactttttattcttttatagaatgtagaaggcaaagcataaaaataattataaatccatgctaatcagtagacaatatatcaaggtgtagtttgtgatattacaaatgcaatttatgacacatataacaatatgactgaatcttgaggatattatgctaagtgaaataagccagttacaaataccatttgatttcatttatatgaggtacgtagaattattaaatgcataaagacagaaagtagaatgatagttgccaacagctggggattggaagaaagagttgttcttaatagacgcagagcttcagtttgggaaacttaaaaagttctgaagaaggattgcccaacaatgtgaatgtacttaacactactggactgtacatttaaaaacagttaacacggtcaactttatgttatgtgtattttatcacaattaaaaaaattttgttaatatgggctttggaaccagatgaccatgaatttgcatttcaagttcttttaactcctagtgaagtggtgttgttgtctggggtaaatacccgggttcattgtcttgcatcaagaagattaaggacgtggacatacatgagaagtgactttaggagcggaatgtaataggcaaaagaaagagaaaggagaacagctctctctcttgcgaaagagaggggcatccaaatgggacttctggcccacgtggagtgtaccagattttataggcaggctggaggaggcggtgtctgatttatgtagggcctgcagattggttggatcaggtgtgatgtttacgtagcacacagggaaggcaggccaccccatcgtaatcttattatgcaaacagcctttccacttggccagtgccatgttgtctgctccttactgtacacctggctggcaaagagaagagaagacagagctgccattttgaacatgcctagttccaggtagccttttcctgttggcacaactgcaggcattcgcctgtgcaagcttctagcttgcttgtctatgtctgcagctcgattttacaggctgctctttgttagaaaagaaaatgattttggggctgcttttcattaaaaggaaaacctttctgaggactccagtaccctcactatctgcctaaataatttcttcttaactcctatatcactagctgagtaaccttaggctaatagccattcactctgagccttttttcctgtaggataaaataaaaataaagttgcaaatgcatgtaaaacccctggggcacagtaaagagaataaacattctagatggcaacctctttgatggcaagtcttaattctaatactactccaaaatgcaaggctaactgtgatttcatttcaggagtgtatttttgcaaatgattatgtaatcaaagattgaggaacaaaaagaagctgcattaaagttgtgactcaggtgactagatgaagactggaatgactttctcacttctgttactgtgcacacattttagaataagacaaagtcagtcttccaaaactaactttttaaaatgttttgggggtggtgtgggagtggaaaagggaaggcagcactaaaagggatatatgaacactgatattttccctccgtgtgaacatactttcataggctgccccatggatggctttgtgatacctcacgcagtttcctttctcatcagcccttcacttgtcctaagggacagcaccccgcaaaaacacactatttcacgtagacctgcagtatccacaaagaaaagatgatctgggacgtcctctgatcttgcgtgtggaggatcctttgccagcttctgcattctctctgtctgcgcaggactgtgaggcatctctgggaagccatcagctctcaggggcaggcacaggaaacagctcttcttgttggcaaaatccagttcggtggtttggaacagggtagacagagaaacaaacaagtgtttgttcataggctgagacctagggggtgtataaggagtaatgatcctatcacctaaggaggatgaattctgggtcattttatgaactgtcttccttagaaaagcctccgaagcaactggcagatgaaaactggaaactattttgagctgggatcagggagtccagggagctcagcagaccaggttactgccactgccactcactaattaagcacatggacaaattgctgccttttcttggcctcttttcctcctcataaacagatgaatccaaaacttttctaaat

SEQ ID NO: 11135 - RNA, 4603 nt, Homo sapiens
  source 1..4603: mol_type = other RNA
ctgaatagctgggactacaggtgcatgccaccacgcccagcttatttttgtatttttagtagagatggggtttcatcgtatcggtcaggctggtcttgaactcctgaccttgtgatccgcccacctcagcctcccaaagtgctggggttacaggcatgagccacagcacccggccgagaagtctcatttttaaaattaaaataaaataggtagatggatggatagataaaacaaaaaatatatgaacttccttgtctcagaggcaaatttgtgttcttaaaagttctgcaggcagaaggacactagatcacagtcacattgcatccccgacttccttagtccatcgcttcccccaaaaatggattaggaatgggcagtctgcgagggaagcatgttggctagggtgggcaaggcagaaagagaaggaaagactcttaaaaagaaaagaaggataaatatcgccagggagtcaagcacaagcaatctttcttattccctcctttccatctgtagcacaaaccccagttaatcaattactttcttgaagagaattactgttacgtggaaagcgacctaagaaagcatttgttgtcagcattatgcactgcaggccttatcacaatcaggccaaaaaagtaccattacagagccaaaggagatcatctaatttcatagaatcccttcttgtgaaagtatgttattggatatgcctgatgctgtcaaagtggggtggaggaaggctgagcagtactaagaatacggctttttttgtggttgttcaaagaagaactatagcaattcttcctttccagtgtttttataatttggtttagaatcagccaagacaaaacaagagaagggctggaaaccttccctccaagaagttggaatcaatatattttcctgaaatattttgttagtgtggtaattaagatagagtttcactcagaactttatgcatttgactatttcctcattaaaaaaaaaaggtcagtgtgctaataaagataaatacattctattttcctttcaggattttaattctctcaaccctatcatagtactcaagagcaagcttacctgatgtccttacaaaatcctggttctaatgctctacagcaaaatcacctgtgcaaatatgtgtgcacactgtgtgtgtgtgtgtgtgtgtgtgtgtgtgtgtcagagtgagagagaatgcattgagcactggcatgtgcatctgaaaagttttagtcttaattcctcattctttatttttggtagcatcattaacattacaaaaacagtaaactggtataggtttcaaacatgcaaacttgctaatagtattctgcagagggacaattccaggatcagagagaatacttcttgctccaaacacaattttacattttgaaatatgatttactttctggattgcagccaggcaattaccattcacaaatatttcaagtgagagagagaaagtggttgctactagtcccataatttggaattgctgctaacagattttacatatcatctacttttctgccattctctttcagaaaatacaattaaaccttaatatttctgcattttaagtcttactgtcagcttcgtcactgcttgaaacaaaagtgtgtaagtggctccctctggtgctgccactagtattaatttttctattcgcaaccacagatgtaacccagagaagcaggaaaaagtaggtagaagccctcataactggaaatgtctcttggcacacaatcccacatggaataatattagataagagatgagggggtttggagggcggggtaggaatagatgcttaatatcttccgtggccttttttcctcacttcatatacacaaaaggaaattgcaaaagctttaagaaaagtcatgtttactaaaccccagccaaaatcccccattcttgttgcctaatactaatgacctaagaaagtacttaagtactacttctaatggaccttgacagggccatcagtcaccagcccagcactccacttgacctggggcctacatagccatgattagagcaaaagtgggatcataaaaagtctcttccaagtggcaaccgagggctccagaacagcacctctgaatggcagtggtgaaggaagctggcaaaacttccttctgtggctgtggtccatagttctctctgatgaccactctttcaatgtaagtcctactcacagacagacaatgtttgaaatttagactccgtaagggaatgatctgacttctaggtcagccaccacagtgtacagtcccaatgattagtttatagcaatctgcaggctctctcatgctgatcttgccctcttttctgccaaagaggcagcacatcttccctgctatatttctctaaagcacagcacagcctccaccaccagccagaatgttaatgcattatcactctgtacactgagaaaacaagtgaccatatgtagcctatgccagcggagctgtaactgtgaagaacaatggctctgagtcaacaacagaattaaactactccctcttgtgaagctcttctgaatattttaagtgttgccttgaaagtgtgggattatgtgcaagcataaacattagcttaatgcaattttttggtacagaatatgccagagtttaaaaatcagaattgaaatgcagaaaataactttgggataaatttaatttttttatgtgtgattaaaacatgattgaagtggcatactttatgtataattaaagttgctttgtaattaagagatttaaacatgtatagaaaatgatacagcctagtttggagattttacaaaggcacctattaaatactcacccctagcaagcctatgactcaaatgttttcacattctaatgctgatagagttcttgaattttctaaagctgccaatttcaccatttctaaatgctttatccctccttccatgtgctagtgaaataaaagcagcccaatctcccctgcattaacaaaaacatggatgtagaacaccatatcttaacttcaaaaactccaggtgaataaagaaggactgtcacaattgaggtagcgtttgactcatctttgccttctccattgtgcctagcaccatgtcccacccagtgcttaggaaatacgtgataaatggctattagtaggtgagcacagtgtgtccgtgtttatgtatggagggttctcatgataatgcaaacacttctgaacatttttatgtgccaggcaaaagtgctatgttattttgtttattcccataacggccctatactttttagagttttagaatagcctggtgaaggaatgacactcaaaatagactagcaggactactctcagtgtattttttacagacagaaaaactaaatcaaagagaggtgaagtccacacagaatcatgaattttagtactaacttagcagcagtaccacctattaagctaaagaattatgcagaacaagtttggttgttttcccccttatcttgctcatttgtgtcacccctttcccagacccaaattcctcaatctcccaccctctccagagattgcctcttggcccccctacaggtccctaaaacatccttctagtaagcacctggcattaacctaggcttgttctcactagcaatgatcttggtttaaactgatcttcctggccttccccatcaatacttgtcttttttatgtttcattctttttagccaagtatcacatggcggagggaaatagtcagacaaacttattcatattagagtgttggttgctgatatttgcatttagaaggcttttgcaacatttcaaaagcacaatggaaaatcctgaatttgggttctggatttaggtacagaaaggatgccatgtaagagacgtgtgtaagagacattgttgactggatacagggatcaggagacaggaaatcaggagttggaaatgggggaaagaaataatattcatgaagataagcaaaaaaatatatggactgatagatgaatgctagatttattttcctgggggccagtgacacgttttctaggggccagtgacacgttttctagtgtttttccacattcccgtctacagtacatatggaatatgaacagttttttccaagaaaagtgattgtttcttctcaggctttctcatatcaatcattcaactataattttcaattaataaagataaacagaggtagatagatacacatttacatattgatatatatgtatacatatggcagttttgcaaacctgagtgtagcaggataaataaaagatattgcaatgttaaagatggctctttatactctttctaacactctaacaaattattccatttccagtgattataccttcgttctcccctatagcagcaccacccatactcttgtttttctcagatttctatggtagagtgtcccacgagaggctgttctgtgagatctcaggcttcctaggggttctagagaaggctcgtgaagaaatgacattcaaaatagcataccaggactattcccagcgtattttgagttacaactggcagagttgtaatgcacctattcttttttttttttttttgagacagagtctcgctctgt

SEQ ID NO: 11136 - RNA, 3655 nt, Homo sapiens
  source 1..3655: mol_type = other RNA
ctgaatagctgggactacaggtgcatgccaccacgcctgactaattaaactattttttttgtagagacagggccttgctatgttgcccaggttggtcttgaacctcctgggcttaagcaattctcctgcgttggcctcccaaagtactgggattacaggcatgagccactgcacctggcctacatttttatttcagttgtcgtgtctctcaggctctaaacaatttccagcccaaaccacagcaccatcctgatgaaaagggccagatattaagacagctgttaggcagttaacctgtaattaaaaggctgtggcaacttcagttccatgacgacctccgactttaacacagtctcgaggaaatttgtccaattgttcatatgccagccgcccatcttctcccagagacaagagggtttctgaggccacatttctgatttcttcagtatcagattgacacaatgtcaccagcattttaatgctttcagtagcctcaaggattttcagagccaggcaagctgctttctggagctggaggtttgtctttgttagtgcttcacagtaatagagcaaggccttttccctgaaatgctgatttttggaggctgctgccaagtaaagcgtcacagcctcactaacttcgttgtcctctctggttaatagcagagccagagtcctgagtacttcctgctgggccaggaggttgctgggagcaaggtcactcatggtttgtagcagtttttcatctcttagtgattgcagagtctgaaccatggaaacttgcctggccagctggctcaggtaactctccaggtcactgacgccgtggctggtgaagtaactgtaatactggaaaacagtgacgacttccgaggacaggctggaggaaagcagaggctcagcccggtccagaatttgggacaccagggttcgaaacactgggtctgcaagtcctggatattctttgttgacagttctggcaaagctggcctccagctgcttcatcactctgtccgctgggctgtggtagacaccaacagggctgcagcacttggtccagaatgacagcaaagacagctttttgtgaaattctggtatggcttccacaacagaactgatatttcctatgttctcatcactgacagctgcgagtttctccatcacttggatctgcctagaaagcttctctaagagacttcttgccacaaatggggttttgcttgagaaaacaatttgctgcacgagttgggtgcagtactggaggtgcctgacgatggtgatgtccaggctctcgttgcctgtggtcagtgggagaggacttcctgccacactggtcccaactcctgtgtcttcagtgagcgcttcactgagatgccccctggcttctgggtgaaccgacctgtaactgtgtttctcagtctcagtgtctgaaaatactgagtcagcacctccgccaacattacaaacctcatcaccatcctcctcctcgtcaaaatcagaggtgttcaggaaatcaaagctttctaaagcactttcaactgtgagacttaaactggaagacctgctgcggcttactgctggcttgcattttagaatatcatccaaattcatgacttcttggttcagatcctgaaactctttatactgctctttatgtggttctaatgcaagtaaaagcccattaaaagcatcctctaagcttccatctagaaaggatctgcagccttcagattctccaccaacagaaccctcagagagcagcctgtctgtggccattggcacctctgcagatgtgagcctcttgaccagctgctttgtgatgtttccttccgaagtgtccagttccacaggcttgagctcagaggcctcctcagactcttgcagaagtgcttctgcaacatcattctcaaggaacaggtgctcagccccagcacctgaggactgtcggcggcaagcctcagatggggccgaggcaggttttctgggctcctctgggtcttcctccttcaggtgtgactttggctcttggccttctcccagggagttcctggaagatgctgagctggtgtcatccataccctcattctgggaggccaagctgctgaggttaaactccgcaggggtgatggtaatttctggatttgttgagttggaaggggagcctgttgagtgggaggtgagggcgcagtccccgttgggcaggtcactgaagctgagcgacagtggcattttctcctcggctgcctttccattttcaaagatgtcatcaggtagatttgaaaagaaggagtggtctttgaaggtgggcgtttccggggtaccctggctgtacatggacattctcctctgaagggctgctgccttgttcccagcgcctgaggatgcggtcatgtcctccacgtcaaatggataccaggtgatttccaggttcagtttgatggtaccaaggtcattgatgtcgacagccactacctgaggtcgggctgcaaacagctctttggtctcacaggtcacgctacctaccaggatgtgagttgctagccctttgagctccgtgaccttgatggagatgaacccaactatcaggggcagaaaaactgtttcttctccatcccagctctgcttgccatttacttctattttgcctttcagtttccaccgctgccggccatacttcatgaaaatttcatattgatctccaggacagaggcgtgcaaagccagccagacctttcatcttgatggagaattctcccagcagattctctagctccacttcaatggtgcacatattctctgtgtactccttgaagctccgattgatctctgtcagactctcccgggcagctttgctggcaggggatgttgcgaaggcttgcttcattttgctggcaccatcctggaggcgtcgctggatacaataagcttcatagagttcatctaccttacttatatgaaactccaggcgtctcatgtatctttcaattgttttaatttgcttgtctaggtcatacagtacacccaggcgagagtttcttttcatatcttttaactgagctgtcaacttgtccagctccgtctggtgaacctccagatattcatcaagtccatttttcaaggccctgtagacttcttccacccttttaggctgaggctctttggggggattgttgtttttgtggcctaaattgtgcattttcttcagtttggcctgaggcttcttgagagcggaggaattttcaatgaaggagttacacctggatcgcctttcctggaggccgctgaaacccgcaaaggactggcttctaatgatcccattgggccctccaggcgaaaaagactgggatcctaccaacatgatttccgggagtctggtcggtagtcatgatctgatttgtctgtcaacaagaatccaacagttcaggctcttgacacgtccctcttcagcctagggtgtgcagatgttatggaatcatcaccctcatagtcagccaagcacatcctcatttcagggtcccagaaactagcacctggcacagcctggaccatatgaccaccacctggtgagccgtttgctcccacacgtgaattctgttctgttcttgaaagcaggataggaacctacactgtgcatggcccttcttttttcctttttt

SEQ ID NO: 11137 - RNA, 3490 nt, Homo sapiens
  source 1..3490: mol_type = other RNA
ctgaatagctgggactacaggtgcatgccaccacgcctgactaattaaactattttttttgtagagacagggccttgctatgttgcccaggttggtcttgaacctcctgggcttaagcaattctcctgcgttggcctcccaaagtactgggattacaggcatgagccactgcacctggcctacatttttatttcagttgtcgtgtctctcaggctctaaacaatttccagcccaaaccacagcaccatcctgatgaaaagggccagatattaagacagctgttaggcagttaacctgtaattaaaaggctgtggcaacttcagttccatgacgacctccgactttaacacagtctcgaggaaatttgtccaattgttcatatgccagccgcccatcttctcccagagacaagagggtttctgaggccacatttctgatttcttcagtatcagattgacacaatgtcaccagcattttaatgctttcagtagcctcaaggattttcagagccaggcaagctgctttctggagctggaggtttgtctttgttagtgcttcacagtaatagagcaaggccttttccctgaaatgctgatttttggaggctgctgccaagtaaagcgtcacagcctcactaacttcgttgtcctctctggttaatagcagagccagagtcctgagtacttcctgctgggccaggaggttgctgggagcaaggtcactcatggtttgtagcagtttttcatctcttagtgattgcagagtctgaaccatggaaacttgcctggccagctggctcaggtaactctccaggtcactgacgccgtggctggtgaagtaactgtaatactggaaaacagtgacgacttccgaggacaggctggaggaaagcagaggctcagcccggtccagaatttgggacaccagggttcgaaacactgggtctgcaagtcctggatattctttgttgacagttctggcaaagctggcctccagctgcttcatcactctgtccgctgggctgtggtagacaccaacagggctgcagcacttggtccagaatgacagcaaagacagctttttgtgaaattctggtatggcttccacaacagaactgatatttcctatgttctcatcactgacagctgcgagtttctccatcacttggatctgcctagaaagcttctctaagagacttcttgccacaaatggggttttgcttgagaaaacaatttgctgcacgagttgggtgcagtactggaggtgcctgacgatggtgatgtccaggctctcgttgcctgtggtcagtgggagaggacttcctgccacactggtcccaactcctgtgtcttcagtgagcgcttcactgagatgccccctggcttctgggtgaaccgacctgtaactgtgtttctcagtctcagtgtctgaaaatactgagtcagcacctccgccaacattacaaacctcatcaccatcctcctcctcgtcaaaatcagaggtgttcaggaaatcaaagctttctaaagcactttcaactgtgagacttaaactggaagacctgctgcggcttactgctggcttgcattttagaatatcatccaaattcatgacttcttggttcagatcctgaaactctttatactgctctttatgtggttctaatgcaagtaaaagcccattaaaagcatcctctaagcttccatctagaaaggatctgcagccttcagattctccaccaacagaaccctcagagagcagcctgtctgtggccattggcacctctgcagatgtgagcctcttgaccagctgctttgtgatgtttccttccgaagtgtccagttccacaggcttgagctcagaggcctcctcagactcttgcagaagtgcttctgcaacatcattctcaaggaacaggtgctcagccccagcacctgaggactgtcggcggcaagcctcagatggggccgaggcaggttttctgggctcctctgggtcttcctccttcaggtgtgactttggctcttggccttctcccagggagttcctggaagatgctgagctggtgtcatccataccctcattctgggaggccaagctgctgaggttaaactccgcaggggtgatggtaatttctggatttgttgagttggaaggggagcctgttgagtgggaggtgagggcgcagtccccgttgggcaggtcactgaagctgagcgacagtggcattttctcctcggctgcctttccattttcaaagatgtcatcaggtagatttgaaaagaaggagtggtctttgaaggtgggcgtttccggggtaccctggctgtacatggacattctcctctgaagggctgctgccttgttcccagcgcctgaggatgcggtcatgtcctccacgtcaaatggataccaggtgatttccaggttcagtttgatggtaccaaggtcattgatgtcgacagccactacctgaggtcgggctgcaaacagctctttggtctcacaggtcacgctacctaccaggatgtgagttgctagccctttgagctccgtgaccttgatggagatgaacccaactatcaggggcagaaaaactgtttcttctccatcccagctctgcttgccatttacttctattttgcctttcagtttccaccgctgccggccatacttcatgaaaatttcatattgatctccaggacagaggcgtgcaaagccagccagacctttcatcttgatggagaattctcccagcagattctctagctccacttcaatggtgcacatattctctgtgtactccttgaagctccgattgatctctgtcagactctcccgggcagctttgctggcaggggatgttgcgaaggcttgcttcattttgctggcaccatcctggaggcgtcgctggatacaataagcttcatagagttcatctaccttacttatatgaaactccaggcgtctcatgtatctttcaattgttttaatttgcttgtctaggtcatacagtacacccaggcgagagtttcttttcatatcttttaactgagctgtcaacttgtccagctccgtctggtgaacctccagatattcatcaagtccatttttcaaggccctgtagacttcttccacccttttaggctgaggctctttggggggattgttgtttttgtggcctaaattgtgcattttcttcagtttggcctgaggcttcttgagagcggaggaattttcaatgaaggagttacacctggatcgcctttcctggaggccgctgaaacccgcaaaggactggcttctaatgatcccattgggccctccaggcgaaaaagactgggatcctaccaacatgatttccgggagtctggtcggtagtccaccacctggtgagccgtttgctcccacacgtgaattctgttctgttcttgaaagcaggataggaacctacactgtgcatggcccttcttttttccttttttcaatt

SEQ ID NO: 11138 - RNA, 3793 nt, Homo sapiens
  source 1..3793: mol_type = other RNA
ctgaatagctgggactacaggtgcatgccaccacgcctgactaattaaactattttttttgtagagacagggccttgctatgttgcccaggttggtcttgaacctcctgggcttaagcaattctcctgcgttggcctcccaaagtactgggattacaggcatgagccactgcacctggcctacatttttatttcagttgtcgtgtctctcaggctctaaacaatttccagcccaaaccacagcaccatcctgatgaaaagggccagatattaagacagctgttaggcagttaacctgtaattaaaaggctgtggcaacttcagttccatgacgacctccgactttaacacagtctcgaggaaatttgtccaattgttcatatgccagccgcccatcttctcccagagacaagagggtttctgaggccacatttctgatttcttcagtatcagattgacacaatgtcaccagcattttaatgctttcagtagcctcaaggattttcagagccaggcaagctgctttctggagctggaggtttgtctttgttagtgcttcacagtaatagagcaaggccttttccctgaaatgctgatttttggaggctgctgccaagtaaagcgtcacagcctcactaacttcgttgtcctctctggttaatagcagagccagagtcctgagtacttcctgctgggccaggaggttgctgggagcaaggtcactcatggtttgtagcagtttttcatctcttagtgattgcagagtctgaaccatggaaacttgcctggccagctggctcaggtaactctccaggtcactgacgccgtggctggtgaagtaactgtaatactggaaaacagtgacgacttccgaggacaggctggaggaaagcagaggctcagcccggtccagaatttgggacaccagggttcgaaacactgggtctgcaagtcctggatattctttgttgacagttctggcaaagctggcctccagctgcttcatcactctgtccgctgggctgtggtagacaccaacagggctgcagcacttggtccagaatgacagcaaagacagctttttgtgaaattctggtatggcttccacaacagaactgatatttcctatgttctcatcactgacagctgcgagtttctccatcacttggatctgcctagaaagcttctctaagagacttcttgccacaaatggggttttgcttgagaaaacaatttgctgcacgagttgggtgcagtactggaggtgcctgacgatggtgatgtccaggctctcgttgcctgtggtcagtgggagaggacttcctgccacactggtcccaactcctgtgtcttcagtgagcgcttcactgagatgccccctggcttctgggtgaaccgacctgtaactgtgtttctcagtctcagtgtctgaaaatactgagtcagcacctccgccaacattacaaacctcatcaccatcctcctcctcgtcaaaatcagaggtgttcaggaaatcaaagctttctaaagcactttcaactgtgagacttaaactggaagacctgctgcggcttactgctggcttgcattttagaatatcatccaaattcatgacttcttggttcagatcctgaaactctttatactgctctttatgtggttctaatgcaagtaaaagcccattaaaagcatcctctaagcttccatctagaaaggatctgcagccttcagattctccaccaacagaaccctcagagagcagcctgtctgtggccattggcacctctgcagatgtgagcctcttgaccagctgctttgtgatgtttccttccgaagtgtccagttccacaggcttgagctcagaggcctcctcagactcttgcagaagtgcttctgcaacatcattctcaaggaacaggtgctcagccccagcacctgaggactgtcggcggcaagcctcagatggggccgaggcaggttttctgggctcctctgggtcttcctccttcaggtgtgactttggctcttggccttctcccagggagttcctggaagatgctgagctggtgtcatccataccctcattctgggaggccaagctgctgaggttaaactccgcaggggtgatggtaatttctggatttgttgagttggaaggggagcctgttgagtgggaggtgagggcgcagtccccgttgggcaggtcactgaagctgagcgacagtggcattttctcctcggctgcctttccattttcaaagatgtcatcaggtagatttgaaaagaaggagtggtctttgaaggtgggcgtttccggggtaccctggctgtacatggacattctcctctgaagggctgctgccttgttcccagcgcctgaggatgcggtcatgtcctccacgtcaaatggataccaggtgatttccaggttcagtttgatggtaccaaggtcattgatgtcgacagccactacctgaggtcgggctgcaaacagctctttggtctcacaggtcacgctacctaccaggatgtgagttgctagccctttgagctccgtgaccttgatggagatgaacccaactatcaggggcagaaaaactgtttcttctccatcccagctctgcttgccatttacttctattttgcctttcagtttccaccgctgccggccatacttcatgaaaatttcatattgatctccaggacagaggcgtgcaaagccagccagacctttcatcttgatggagaattctcccagcagattctctagctccacttcaatggtgcacatattctctgtgtactccttgaagctccgattgatctctgtcagactctcccgggcagctttgctggcaggggatgttgcgaaggcttgcttcattttgctggcaccatcctggaggcgtcgctggatacaataagcttcatagagttcatctaccttacttatatgaaactccaggcgtctcatgtatctttcaattgttttaatttgcttgtctaggtcatacagtacacccaggcgagagtttcttttcatatcttttaactgagctgtcaacttgtccagctccgtctggtgaacctccagatattcatcaagtccatttttcaaggccctgtagacttcttccacccttttaggctgaggctctttggggggattgttgtttttgtggcctaaattgtgcattttcttcagtttggcctgaggcttcttgagagcggaggaattttcaatgaaggagttacacctggatcgcctttcctggaggccgctgaaacccgcaaaggactggcttctaatgatcccattgggccctccaggcgaaaaagactgggatcctaccaacatgatttccgggagtctggtcggtagtccattgtcttagcaggtgacttcaatccagagagggggacaggctagcaggaaaaagggtaaatagttactgcccagattgaagactccaaagtgggcagacaacaaatcggtatgtttgcagagtgtcgacaattgccctttaaagactcaaagaaagaaaagctaaaaaaaacaacagcagcagaactctctggtagtacatccagatgtaatggaaagaccaatttcactagaccttcctcaaagctacgcgaagcagctcagcaaggaaggcagtttgagcgagttacttccccagagagagaaggacaaacagcctcctcccccatgttgctgcaggtttttaaatcccctccctccctctccaggagagagcagccctggagtttgtatgcattcttgcgaggta

SEQ ID NO: 11139 - RNA, 3614 nt, Homo sapiens
  source 1..3614: mol_type = other RNA
ctgaatagctgggactacaggtgcatgccaccacgcctgactaattaaactattttttttgtagagacagggccttgctatgttgcccaggttggtcttgaacctcctgggcttaagcaattctcctgcgttggcctcccaaagtactgggattacaggcatgagccactgcacctggcctacatttttatttcagttgtcgtgtctctcaggctctaaacaatttccagcccaaaccacagcaccatcctgatgaaaagggccagatattaagacagctgttaggcagttaacctgtaattaaaaggctgtggcaacttcagttccatgacgacctccgactttaacacagtctcgaggaaatttgtccaattgttcatatgccagccgcccatcttctcccagagacaagagggtttctgaggccacatttctgatttcttcagtatcagattgacacaatgtcaccagcattttaatgctttcagtagcctcaaggattttcagagccaggcaagctgctttctggagctggaggtttgtctttgttagtgcttcacagtaatagagcaaggccttttccctgaaatgctgatttttggaggctgctgccaagtaaagcgtcacagcctcactaacttcgttgtcctctctggttaatagcagagccagagtcctgagtacttcctgctgggccaggaggttgctgggagcaaggtcactcatggtttgtagcagtttttcatctcttagtgattgcagagtctgaaccatggaaacttgcctggccagctggctcaggtaactctccaggtcactgacgccgtggctggtgaagtaactgtaatactggaaaacagtgacgacttccgaggacaggctggaggaaagcagaggctcagcccggtccagaatttgggacaccagggttcgaaacactgggtctgcaagtcctggatattctttgttgacagttctggcaaagctggcctccagctgcttcatcactctgtccgctgggctgtggtagacaccaacagggctgcagcacttggtccagaatgacagcaaagacagctttttgtgaaattctggtatggcttccacaacagaactgatatttcctatgttctcatcactgacagctgcgagtttctccatcacttggatctgcctagaaagcttctctaagagacttcttgccacaaatggggttttgcttgagaaaacaatttgctgcacgagttgggtgcagtactggaggtgcctgacgatggtgatgtccaggctctcgttgcctgtggtcagtgggagaggacttcctgccacactggtcccaactcctgtgtcttcagtgagcgcttcactgagatgccccctggcttctgggtgaaccgacctgtaactgtgtttctcagtctcagtgtctgaaaatactgagtcagcacctccgccaacattacaaacctcatcaccatcctcctcctcgtcaaaatcagaggtgttcaggaaatcaaagctttctaaagcactttcaactgtgagacttaaactggaagacctgctgcggcttactgctggcttgcattttagaatatcatccaaattcatgacttcttggttcagatcctgaaactctttatactgctctttatgtggttctaatgcaagtaaaagcccattaaaagcatcctctaagcttccatctagaaaggatctgcagccttcagattctccaccaacagaaccctcagagagcagcctgtctgtggccattggcacctctgcagatgtgagcctcttgaccagctgctttgtgatgtttccttccgaagtgtccagttccacaggcttgagctcagaggcctcctcagactcttgcagaagtgcttctgcaacatcattctcaaggaacaggtgctcagccccagcacctgaggactgtcggcggcaagcctcagatggggccgaggcaggttttctgggctcctctgggtcttcctccttcaggtgtgactttggctcttggccttctcccagggagttcctggaagatgctgagctggtgtcatccataccctcattctgggaggccaagctgctgaggttaaactccgcaggggtgatggtaatttctggatttgttgagttggaaggggagcctgttgagtgggaggtgagggcgcagtccccgttgggcaggtcactgaagctgagcgacagtggcattttctcctcggctgcctttccattttcaaagatgtcatcaggtagatttgaaaagaaggagtggtctttgaaggtgggcgtttccggggtaccctggctgtacatggacattctcctctgaagggctgctgccttgttcccagcgcctgaggatgcggtcatgtcctccacgtcaaatggataccaggtgatttccaggttcagtttgatggtaccaaggtcattgatgtcgacagccactacctgaggtcgggctgcaaacagctctttggtctcacaggtcacgctacctaccaggatgtgagttgctagccctttgagctccgtgaccttgatggagatgaacccaactatcaggggcagaaaaactgtttcttctccatcccagctctgcttgccatttacttctattttgcctttcagtttccaccgctgccggccatacttcatgaaaatttcatattgatctccaggacagaggcgtgcaaagccagccagacctttcatcttgatggagaattctcccagcagattctctagctccacttcaatggtgcacatattctctgtgtactccttgaagctccgattgatctctgtcagactctcccgggcagctttgctggcaggggatgttgcgaaggcttgcttcattttgctggcaccatcctggaggcgtcgctggatacaataagcttcatagagttcatctaccttacttatatgaaactccaggcgtctcatgtatctttcaattgttttaatttgcttgtctaggtcatacagtacacccaggcgagagtttcttttcatatcttttaactgagctgtcaacttgtccagctccgtctggtgaacctccagatattcatcaagtccatttttcaaggccctgtagacttcttccacccttttaggctgaggctctttggggggattgttgtttttgtggcctaaattgtgcattttcttcagtttggcctgaggcttcttgagagcggaggaattttcaatgaaggagttacacctggatcgcctttcctggaggccgctgaaacccgcaaaggactggcttctaatgatcccattgggccctccaggcgaaaaagactgggatcctaccaacatgatttccgggagtctggtcggtagtcctaacgacgacggctccttgtcatgtcaggggcacactcagggttctctggcatataaaagcctccgcaccaatgcaatgcccggagctgcccgcacctccggctttgcagacagcctgagctggctcacttgggtgaaggggaccccgggaggaagtcgggtggacgcgagctgtccccagcgccggctgccctgccgcgtccgctcgcagcagctgcggcgcgcggggt

SEQ ID NO: 11140 - RNA, 3527 nt, Homo sapiens
  source 1..3527: mol_type = other RNA
ctgaatagctgggactacaggtgcatgccaccacgcctgactaattaaactattttttttgtagagacagggccttgctatgttgcccaggttggtcttgaacctcctgggcttaagcaattctcctgcgttggcctcccaaagtactgggattacaggcatgagccactgcacctggcctacatttttatttcagttgtcgtgtctctcaggctctaaacaatttccagcccaaaccacagcaccatcctgatgaaaagggccagatattaagacagctgttaggcagttaacctgtaattaaaaggctgtggcaacttcagttccatgacgacctccgactttaacacagtctcgaggaaatttgtccaattgttcatatgccagccgcccatcttctcccagagacaagagggtttctgaggccacatttctgatttcttcagtatcagattgacacaatgtcaccagcattttaatgctttcagtagcctcaaggattttcagagccaggcaagctgctttctggagctggaggtttgtctttgttagtgcttcacagtaatagagcaaggccttttccctgaaatgctgatttttggaggctgctgccaagtaaagcgtcacagcctcactaacttcgttgtcctctctggttaatagcagagccagagtcctgagtacttcctgctgggccaggaggttgctgggagcaaggtcactcatggtttgtagcagtttttcatctcttagtgattgcagagtctgaaccatggaaacttgcctggccagctggctcaggtaactctccaggtcactgacgccgtggctggtgaagtaactgtaatactggaaaacagtgacgacttccgaggacaggctggaggaaagcagaggctcagcccggtccagaatttgggacaccagggttcgaaacactgggtctgcaagtcctggatattctttgttgacagttctggcaaagctggcctccagctgcttcatcactctgtccgctgggctgtggtagacaccaacagggctgcagcacttggtccagaatgacagcaaagacagctttttgtgaaattctggtatggcttccacaacagaactgatatttcctatgttctcatcactgacagctgcgagtttctccatcacttggatctgcctagaaagcttctctaagagacttcttgccacaaatggggttttgcttgagaaaacaatttgctgcacgagttgggtgcagtactggaggtgcctgacgatggtgatgtccaggctctcgttgcctgtggtcagtgggagaggacttcctgccacactggtcccaactcctgtgtcttcagtgagcgcttcactgagatgccccctggcttctgggtgaaccgacctgtaactgtgtttctcagtctcagtgtctgaaaatactgagtcagcacctccgccaacattacaaacctcatcaccatcctcctcctcgtcaaaatcagaggtgttcaggaaatcaaagctttctaaagcactttcaactgtgagacttaaactggaagacctgctgcggcttactgctggcttgcattttagaatatcatccaaattcatgacttcttggttcagatcctgaaactctttatactgctctttatgtggttctaatgcaagtaaaagcccattaaaagcatcctctaagcttccatctagaaaggatctgcagccttcagattctccaccaacagaaccctcagagagcagcctgtctgtggccattggcacctctgcagatgtgagcctcttgaccagctgctttgtgatgtttccttccgaagtgtccagttccacaggcttgagctcagaggcctcctcagactcttgcagaagtgcttctgcaacatcattctcaaggaacaggtgctcagccccagcacctgaggactgtcggcggcaagcctcagatggggccgaggcaggttttctgggctcctctgggtcttcctccttcaggtgtgactttggctcttggccttctcccagggagttcctggaagatgctgagctggtgtcatccataccctcattctgggaggccaagctgctgaggttaaactccgcaggggtgatggtaatttctggatttgttgagttggaaggggagcctgttgagtgggaggtgagggcgcagtccccgttgggcaggtcactgaagctgagcgacagtggcattttctcctcggctgcctttccattttcaaagatgtcatcaggtagatttgaaaagaaggagtggtctttgaaggtgggcgtttccggggtaccctggctgtacatggacattctcctctgaagggctgctgccttgttcccagcgcctgaggatgcggtcatgtcctccacgtcaaatggataccaggtgatttccaggttcagtttgatggtaccaaggtcattgatgtcgacagccactacctgaggtcgggctgcaaacagctctttggtctcacaggtcacgctacctaccaggatgtgagttgctagccctttgagctccgtgaccttgatggagatgaacccaactatcaggggcagaaaaactgtttcttctccatcccagctctgcttgccatttacttctattttgcctttcagtttccaccgctgccggccatacttcatgaaaatttcatattgatctccaggacagaggcgtgcaaagccagccagacctttcatcttgatggagaattctcccagcagattctctagctccacttcaatggtgcacatattctctgtgtactccttgaagctccgattgatctctgtcagactctcccgggcagctttgctggcaggggatgttgcgaaggcttgcttcattttgctggcaccatcctggaggcgtcgctggatacaataagcttcatagagttcatctaccttacttatatgaaactccaggcgtctcatgtatctttcaattgttttaatttgcttgtctaggtcatacagtacacccaggcgagagtttcttttcatatcttttaactgagctgtcaacttgtccagctccgtctggtgaacctccagatattcatcaagtccatttttcaaggccctgtagacttcttccacccttttaggctgaggctctttggggggattgttgtttttgtggcctaaattgtgcattttcttcagtttggcctgaggcttcttgagagcggaggaattttcaatgaaggagttacacctggatcgcctttcctggaggccgctgaaacccgcaaaggactggcttctaatgatcccattgggccctccaggcgaaaaagactgggatcctaccaacatgatttccgggagtctggtcggtagtcctcataatccctactgcttggtcacagtgtagcatttccacagcagttctccttggcctggagagggtaacagcttctcctttatgttcaccattcaccccctgtactggatttttctccaccttgtcgcctcctctccaggtt

SEQ ID NO: 11141 - RNA, 3506 nt, Homo sapiens
  source 1..3506: mol_type = other RNA
ctgaatagctgggactacaggtgcatgccaccacgcctgactaattaaactattttttttgtagagacagggccttgctatgttgcccaggttggtcttgaacctcctgggcttaagcaattctcctgcgttggcctcccaaagtactgggattacaggcatgagccactgcacctggcctacatttttatttcagttgtcgtgtctctcaggctctaaacaatttccagcccaaaccacagcaccatcctgatgaaaagggccagatattaagacagctgttaggcagttaacctgtaattaaaaggctgtggcaacttcagttccatgacgacctccgactttaacacagtctcgaggaaatttgtccaattgttcatatgccagccgcccatcttctcccagagacaagagggtttctgaggccacatttctgatttcttcagtatcagattgacacaatgtcaccagcattttaatgctttcagtagcctcaaggattttcagagccaggcaagctgctttctggagctggaggtttgtctttgttagtgcttcacagtaatagagcaaggccttttccctgaaatgctgatttttggaggctgctgccaagtaaagcgtcacagcctcactaacttcgttgtcctctctggttaatagcagagccagagtcctgagtacttcctgctgggccaggaggttgctgggagcaaggtcactcatggtttgtagcagtttttcatctcttagtgattgcagagtctgaaccatggaaacttgcctggccagctggctcaggtaactctccaggtcactgacgccgtggctggtgaagtaactgtaatactggaaaacagtgacgacttccgaggacaggctggaggaaagcagaggctcagcccggtccagaatttgggacaccagggttcgaaacactgggtctgcaagtcctggatattctttgttgacagttctggcaaagctggcctccagctgcttcatcactctgtccgctgggctgtggtagacaccaacagggctgcagcacttggtccagaatgacagcaaagacagctttttgtgaaattctggtatggcttccacaacagaactgatatttcctatgttctcatcactgacagctgcgagtttctccatcacttggatctgcctagaaagcttctctaagagacttcttgccacaaatggggttttgcttgagaaaacaatttgctgcacgagttgggtgcagtactggaggtgcctgacgatggtgatgtccaggctctcgttgcctgtggtcagtgggagaggacttcctgccacactggtcccaactcctgtgtcttcagtgagcgcttcactgagatgccccctggcttctgggtgaaccgacctgtaactgtgtttctcagtctcagtgtctgaaaatactgagtcagcacctccgccaacattacaaacctcatcaccatcctcctcctcgtcaaaatcagaggtgttcaggaaatcaaagctttctaaagcactttcaactgtgagacttaaactggaagacctgctgcggcttactgctggcttgcattttagaatatcatccaaattcatgacttcttggttcagatcctgaaactctttatactgctctttatgtggttctaatgcaagtaaaagcccattaaaagcatcctctaagcttccatctagaaaggatctgcagccttcagattctccaccaacagaaccctcagagagcagcctgtctgtggccattggcacctctgcagatgtgagcctcttgaccagctgctttgtgatgtttccttccgaagtgtccagttccacaggcttgagctcagaggcctcctcagactcttgcagaagtgcttctgcaacatcattctcaaggaacaggtgctcagccccagcacctgaggactgtcggcggcaagcctcagatggggccgaggcaggttttctgggctcctctgggtcttcctccttcaggtgtgactttggctcttggccttctcccagggagttcctggaagatgctgagctggtgtcatccataccctcattctgggaggccaagctgctgaggttaaactccgcaggggtgatggtaatttctggatttgttgagttggaaggggagcctgttgagtgggaggtgagggcgcagtccccgttgggcaggtcactgaagctgagcgacagtggcattttctcctcggctgcctttccattttcaaagatgtcatcaggtagatttgaaaagaaggagtggtctttgaaggtgggcgtttccggggtaccctggctgtacatggacattctcctctgaagggctgctgccttgttcccagcgcctgaggatgcggtcatgtcctccacgtcaaatggataccaggtgatttccaggttcagtttgatggtaccaaggtcattgatgtcgacagccactacctgaggtcgggctgcaaacagctctttggtctcacaggtcacgctacctaccaggatgtgagttgctagccctttgagctccgtgaccttgatggagatgaacccaactatcaggggcagaaaaactgtttcttctccatcccagctctgcttgccatttacttctattttgcctttcagtttccaccgctgccggccatacttcatgaaaatttcatattgatctccaggacagaggcgtgcaaagccagccagacctttcatcttgatggagaattctcccagcagattctctagctccacttcaatggtgcacatattctctgtgtactccttgaagctccgattgatctctgtcagactctcccgggcagctttgctggcaggggatgttgcgaaggcttgcttcattttgctggcaccatcctggaggcgtcgctggatacaataagcttcatagagttcatctaccttacttatatgaaactccaggcgtctcatgtatctttcaattgttttaatttgcttgtctaggtcatacagtacacccaggcgagagtttcttttcatatcttttaactgagctgtcaacttgtccagctccgtctggtgaacctccagatattcatcaagtccatttttcaaggccctgtagacttcttccacccttttaggctgaggctctttggggggattgttgtttttgtggcctaaattgtgcattttcttcagtttggcctgaggcttcttgagagcggaggaattttcaatgaaggagttacacctggatcgcctttcctggaggccgctgaaacccgcaaaggactggcttctaatgatcccattgggccctccaggcgaaaaagactgggatcctaccaacatgatttccgggagtctggtcggtagtccttcaccaaaaacatcatcctcttcatcgaccaggagctcctcagcatcaaaaaactgcatcttggagaggacaggcgcgagaagcagcaggcagcagccccggcagtctcagcagtcacact

SEQ ID NO: 11142 - RNA, 4324 nt, Homo sapiens
  source 1..4324: mol_type = other RNA
ctgaatagctgggactacaggtgcatgccaccacgcctgactaattaaactattttttttgtagagacagggccttgctatgttgcccaggttggtcttgaacctcctgggcttaagcaattctcctgcgttggcctcccaaagtactgggattacaggcatgagccactgcacctggcctacatttttatttcagttgtcgtgtctctcaggctctaaacaatttccagcccaaaccacagcaccatcctgatgaaaagggccagatattaagacagctgttaggcagttaacctgtaattaaaaggctgtggcaacttcagttccatgacgacctccgactttaacacagtctcgaggaaatttgtccaattgttcatatgccagccgcccatcttctcccagagacaagagggtttctgaggccacatttctgatttcttcagtatcagattgacacaatgtcaccagcattttaatgctttcagtagcctcaaggattttcagagccaggcaagctgctttctggagctggaggtttgtctttgttagtgcttcacagtaatagagcaaggccttttccctgaaatgctgatttttggaggctgctgccaagtaaagcgtcacagcctcactaacttcgttgtcctctctggttaatagcagagccagagtcctgagtacttcctgctgggccaggaggttgctgggagcaaggtcactcatggtttgtagcagtttttcatctcttagtgattgcagagtctgaaccatggaaacttgcctggccagctggctcaggtaactctccaggtcactgacgccgtggctggtgaagtaactgtaatactggaaaacagtgacgacttccgaggacaggctggaggaaagcagaggctcagcccggtccagaatttgggacaccagggttcgaaacactgggtctgcaagtcctggatattctttgttgacagttctggcaaagctggcctccagctgcttcatcactctgtccgctgggctgtggtagacaccaacagggctgcagcacttggtccagaatgacagcaaagacagctttttgtgaaattctggtatggcttccacaacagaactgatatttcctatgttctcatcactgacagctgcgagtttctccatcacttggatctgcctagaaagcttctctaagagacttcttgccacaaatggggttttgcttgagaaaacaatttgctgcacgagttgggtgcagtactggaggtgcctgacgatggtgatgtccaggctctcgttgcctgtggtcagtgggagaggacttcctgccacactggtcccaactcctgtgtcttcagtgagcgcttcactgagatgccccctggcttctgggtgaaccgacctgtaactgtgtttctcagtctcagtgtctgaaaatactgagtcagcacctccgccaacattacaaacctcatcaccatcctcctcctcgtcaaaatcagaggtgttcaggaaatcaaagctttctaaagcactttcaactgtgagacttaaactggaagacctgctgcggcttactgctggcttgcattttagaatatcatccaaattcatgacttcttggttcagatcctgaaactctttatactgctctttatgtggttctaatgcaagtaaaagcccattaaaagcatcctctaagcttccatctagaaaggatctgcagccttcagattctccaccaacagaaccctcagagagcagcctgtctgtggccattggcacctctgcagatgtgagcctcttgaccagctgctttgtgatgtttccttccgaagtgtccagttccacaggcttgagctcagaggcctcctcagactcttgcagaagtgcttctgcaacatcattctcaaggaacaggtgctcagccccagcacctgaggactgtcggcggcaagcctcagatggggccgaggcaggttttctgggctcctctgggtcttcctccttcaggtgtgactttggctcttggccttctcccagggagttcctggaagatgctgagctggtgtcatccataccctcattctgggaggccaagctgctgaggttaaactccgcaggggtgatggtaatttctggatttgttgagttggaaggggagcctgttgagtgggaggtgagggcgcagtccccgttgggcaggtcactgaagctgagcgacagtggcattttctcctcggctgcctttccattttcaaagatgtcatcaggtagatttgaaaagaaggagtggtctttgaaggtgggcgtttccggggtaccctggctgtacatggacattctcctctgaagggctgctgccttgttcccagcgcctgaggatgcggtcatgtcctccacgtcaaatggataccaggtgatttccaggttcagtttgatggtaccaaggtcattgatgtcgacagccactacctgaggtcgggctgcaaacagctctttggtctcacaggtcacgctacctaccaggatgtgagttgctagccctttgagctccgtgaccttgatggagatgaacccaactatcaggggcagaaaaactgtttcttctccatcccagctctgcttgccatttacttctattttgcctttcagtttccaccgctgccggccatacttcatgaaaatttcatattgatctccaggacagaggcgtgcaaagccagccagacctttcatcttgatggagaattctcccagcagattctctagctccacttcaatggtgcacatattctctgtgtactccttgaagctccgattgatctctgtcagactctcccgggcagctttgctggcaggggatgttgcgaaggcttgcttcattttgctggcaccatcctggaggcgtcgctggatacaataagcttcatagagttcatctaccttacttatatgaaactccaggcgtctcatgtatctttcaattgttttaatttgcttgtctaggtcatacagtacacccaggcgagagtttcttttcatatcttttaactgagctgtcaacttgtccagctccgtctggtgaacctccagatattcatcaagtccatttttcaaggccctgtagacttcttccacccttttaggctgaggctctttggggggattgttgtttttgtggcctaaattgtgcattttcttcagtttggcctgaggcttcttgagagcggaggaattttcaatgaaggagttacacctggatcgcctttcctggaggccgctgaaacccgcaaaggactggcttctaatgatcccattgggccctccaggcgaaaaagactgggatcctaccaacatgatttccgggagtctggtcggtagtccttcaccaaaaacatcatcctcttcatcgaccaggagctcctcagcatcaaaaaactgcatcttggagaggacaggcgcgagaagcagcaggcagcagccccggcagtctcagcagtcacactgccgaccgaggtgatttcctttccttgggttgcccaagccctctggagggcagcttccgcatctgccctgaagaaagcagtttcattcatatgaataggcttcttgagccttgtgaagagtgaatcccaggtggggtaattctcaccactgaggagaaagaattttttgaagagggctgcagatccggttggatatgaatacagatatcactcaaagtctgaatgcaatgaattctatttcaaagcaacaactttcatatttccttaaagaggaaggtgggtgcttaactttcttgcttatgaatttgaacacaatgggttttgttgaaagagggagttcatatttctcatatcttggttttgcttcaattacaatttatggttgagctggcgcctccggatcctgtccctccatggcctgtttctgatccagtgtaatcgcgaaggtaacaccatggtcccaacagagcggcctaaaacctgctcatggcaaaggaacaaaagggtcttgcagctatcctggaagttaagtccagacgtataaaaatgaaaaagaaaacttaacccccccctttttgttcttttcttaaaaaaaaaaaaaagagtatttgaggcttccgttgacttcttttatcttgtaacttgccttgcctttccttcccttaacttccgactggcccgaaggcagctgctgtgctgggctgccctagcctcctgtgccatgttttatgcatgaagatgatggggcggtaatttattcaagcagagacgatcaccgggctcctgtgtctgccctcgcgtcagaggagccgtgcaat

SEQ ID NO: 11143 - RNA, 3570 nt, Homo sapiens
  source 1..3570: mol_type = other RNA
ctgaatagctgggactacaggtgcatgccaccacgcctgactaattaaactattttttttgtagagacagggccttgctatgttgcccaggttggtcttgaacctcctgggcttaagcaattctcctgcgttggcctcccaaagtactgggattacaggcatgagccactgcacctggcctacatttttatttcagttgtcgtgtctctcaggctctaaacaatttccagcccaaaccacagcaccatcctgatgaaaagggccagatattaagacagctgttaggcagttaacctgtaattaaaaggctgtggcaacttcagttccatgacgacctccgactttaacacagtctcgaggaaatttgtccaattgttcatatgccagccgcccatcttctcccagagacaagagggtttctgaggccacatttctgatttcttcagtatcagattgacacaatgtcaccagcattttaatgctttcagtagcctcaaggattttcagagccaggcaagctgctttctggagctggaggtttgtctttgttagtgcttcacagtaatagagcaaggccttttccctgaaatgctgatttttggaggctgctgccaagtaaagcgtcacagcctcactaacttcgttgtcctctctggttaatagcagagccagagtcctgagtacttcctgctgggccaggaggttgctgggagcaaggtcactcatggtttgtagcagtttttcatctcttagtgattgcagagtctgaaccatggaaacttgcctggccagctggctcaggtaactctccaggtcactgacgccgtggctggtgaagtaactgtaatactggaaaacagtgacgacttccgaggacaggctggaggaaagcagaggctcagcccggtccagaatttgggacaccagggttcgaaacactgggtctgcaagtcctggatattctttgttgacagttctggcaaagctggcctccagctgcttcatcactctgtccgctgggctgtggtagacaccaacagggctgcagcacttggtccagaatgacagcaaagacagctttttgtgaaattctggtatggcttccacaacagaactgatatttcctatgttctcatcactgacagctgcgagtttctccatcacttggatctgcctagaaagcttctctaagagacttcttgccacaaatggggttttgcttgagaaaacaatttgctgcacgagttgggtgcagtactggaggtgcctgacgatggtgatgtccaggctctcgttgcctgtggtcagtgggagaggacttcctgccacactggtcccaactcctgtgtcttcagtgagcgcttcactgagatgccccctggcttctgggtgaaccgacctgtaactgtgtttctcagtctcagtgtctgaaaatactgagtcagcacctccgccaacattacaaacctcatcaccatcctcctcctcgtcaaaatcagaggtgttcaggaaatcaaagctttctaaagcactttcaactgtgagacttaaactggaagacctgctgcggcttactgctggcttgcattttagaatatcatccaaattcatgacttcttggttcagatcctgaaactctttatactgctctttatgtggttctaatgcaagtaaaagcccattaaaagcatcctctaagcttccatctagaaaggatctgcagccttcagattctccaccaacagaaccctcagagagcagcctgtctgtggccattggcacctctgcagatgtgagcctcttgaccagctgctttgtgatgtttccttccgaagtgtccagttccacaggcttgagctcagaggcctcctcagactcttgcagaagtgcttctgcaacatcattctcaaggaacaggtgctcagccccagcacctgaggactgtcggcggcaagcctcagatggggccgaggcaggttttctgggctcctctgggtcttcctccttcaggtgtgactttggctcttggccttctcccagggagttcctggaagatgctgagctggtgtcatccataccctcattctgggaggccaagctgctgaggttaaactccgcaggggtgatggtaatttctggatttgttgagttggaaggggagcctgttgagtgggaggtgagggcgcagtccccgttgggcaggtcactgaagctgagcgacagtggcattttctcctcggctgcctttccattttcaaagatgtcatcaggtagatttgaaaagaaggagtggtctttgaaggtgggcgtttccggggtaccctggctgtacatggacattctcctctgaagggctgctgccttgttcccagcgcctgaggatgcggtcatgtcctccacgtcaaatggataccaggtgatttccaggttcagtttgatggtaccaaggtcattgatgtcgacagccactacctgaggtcgggctgcaaacagctctttggtctcacaggtcacgctacctaccaggatgtgagttgctagccctttgagctccgtgaccttgatggagatgaacccaactatcaggggcagaaaaactgtttcttctccatcccagctctgcttgccatttacttctattttgcctttcagtttccaccgctgccggccatacttcatgaaaatttcatattgatctccaggacagaggcgtgcaaagccagccagacctttcatcttgatggagaattctcccagcagattctctagctccacttcaatggtgcacatattctctgtgtactccttgaagctccgattgatctctgtcagactctcccgggcagctttgctggcaggggatgttgcgaaggcttgcttcattttgctggcaccatcctggaggcgtcgctggatacaataagcttcatagagttcatctaccttacttatatgaaactccaggcgtctcatgtatctttcaattgttttaatttgcttgtctaggtcatacagtacacccaggcgagagtttcttttcatatcttttaactgagctgtcaacttgtccagctccgtctggtgaacctccagatattcatcaagtccatttttcaaggccctgtagacttcttccacccttttaggctgaggctctttggggggattgttgtttttgtggcctaaattgtgcattttcttcagtttggcctgaggcttcttgagagcggaggaattttcaatgaaggagttacacctggatcgcctttcctggaggccgctgaaacccgcaaaggactggcttctaatgatcccattgggccctccaggcgaaaaagactgggatcctaccaacatgatttccgggagtctggtcggtagtccttggcccgttcctccactccccagggcatccttcagttctgcttgcaaaaagtgcgcgtgcccctttcgctcagcaacttcccgaccgtaccctgtgggcttcagatgcccgaacccaccagggtggtggaagctgaggacgctccagtttcaacggctgcttagcattcaacgctcattcaagtc

SEQ ID NO: 11144 - RNA, 3815 nt, Homo sapiens
  source 1..3815: mol_type = other RNA
ctgaatagctgggactacaggtgcatgccaccacgcctgactaattaaactattttttttgtagagacagggccttgctatgttgcccaggttggtcttgaacctcctgggcttaagcaattctcctgcgttggcctcccaaagtactgggattacaggcatgagccactgcacctggcctacatttttatttcagttgtcgtgtctctcaggctctaaacaatttccagcccaaaccacagcaccatcctgatgaaaagggccagatattaagacagctgttaggcagttaacctgtaattaaaaggctgtggcaacttcagttccatgacgacctccgactttaacacagtctcgaggaaatttgtccaattgttcatatgccagccgcccatcttctcccagagacaagagggtttctgaggccacatttctgatttcttcagtatcagattgacacaatgtcaccagcattttaatgctttcagtagcctcaaggattttcagagccaggcaagctgctttctggagctggaggtttgtctttgttagtgcttcacagtaatagagcaaggccttttccctgaaatgctgatttttggaggctgctgccaagtaaagcgtcacagcctcactaacttcgttgtcctctctggttaatagcagagccagagtcctgagtacttcctgctgggccaggaggttgctgggagcaaggtcactcatggtttgtagcagtttttcatctcttagtgattgcagagtctgaaccatggaaacttgcctggccagctggctcaggtaactctccaggtcactgacgccgtggctggtgaagtaactgtaatactggaaaacagtgacgacttccgaggacaggctggaggaaagcagaggctcagcccggtccagaatttgggacaccagggttcgaaacactgggtctgcaagtcctggatattctttgttgacagttctggcaaagctggcctccagctgcttcatcactctgtccgctgggctgtggtagacaccaacagggctgcagcacttggtccagaatgacagcaaagacagctttttgtgaaattctggtatggcttccacaacagaactgatatttcctatgttctcatcactgacagctgcgagtttctccatcacttggatctgcctagaaagcttctctaagagacttcttgccacaaatggggttttgcttgagaaaacaatttgctgcacgagttgggtgcagtactggaggtgcctgacgatggtgatgtccaggctctcgttgcctgtggtcagtgggagaggacttcctgccacactggtcccaactcctgtgtcttcagtgagcgcttcactgagatgccccctggcttctgggtgaaccgacctgtaactgtgtttctcagtctcagtgtctgaaaatactgagtcagcacctccgccaacattacaaacctcatcaccatcctcctcctcgtcaaaatcagaggtgttcaggaaatcaaagctttctaaagcactttcaactgtgagacttaaactggaagacctgctgcggcttactgctggcttgcattttagaatatcatccaaattcatgacttcttggttcagatcctgaaactctttatactgctctttatgtggttctaatgcaagtaaaagcccattaaaagcatcctctaagcttccatctagaaaggatctgcagccttcagattctccaccaacagaaccctcagagagcagcctgtctgtggccattggcacctctgcagatgtgagcctcttgaccagctgctttgtgatgtttccttccgaagtgtccagttccacaggcttgagctcagaggcctcctcagactcttgcagaagtgcttctgcaacatcattctcaaggaacaggtgctcagccccagcacctgaggactgtcggcggcaagcctcagatggggccgaggcaggttttctgggctcctctgggtcttcctccttcaggtgtgactttggctcttggccttctcccagggagttcctggaagatgctgagctggtgtcatccataccctcattctgggaggccaagctgctgaggttaaactccgcaggggtgatggtaatttctggatttgttgagttggaaggggagcctgttgagtgggaggtgagggcgcagtccccgttgggcaggtcactgaagctgagcgacagtggcattttctcctcggctgcctttccattttcaaagatgtcatcaggtagatttgaaaagaaggagtggtctttgaaggtgggcgtttccggggtaccctggctgtacatggacattctcctctgaagggctgctgccttgttcccagcgcctgaggatgcggtcatgtcctccacgtcaaatggataccaggtgatttccaggttcagtttgatggtaccaaggtcattgatgtcgacagccactacctgaggtcgggctgcaaacagctctttggtctcacaggtcacgctacctaccaggatgtgagttgctagccctttgagctccgtgaccttgatggagatgaacccaactatcaggggcagaaaaactgtttcttctccatcccagctctgcttgccatttacttctattttgcctttcagtttccaccgctgccggccatacttcatgaaaatttcatattgatctccaggacagaggcgtgcaaagccagccagacctttcatcttgatggagaattctcccagcagattctctagctccacttcaatggtgcacatattctctgtgtactccttgaagctccgattgatctctgtcagactctcccgggcagctttgctggcaggggatgttgcgaaggcttgcttcattttgctggcaccatcctggaggcgtcgctggatacaataagcttcatagagttcatctaccttacttatatgaaactccaggcgtctcatgtatctttcaattgttttaatttgcttgtctaggtcatacagtacacccaggcgagagtttcttttcatatcttttaactgagctgtcaacttgtccagctccgtctggtgaacctccagatattcatcaagtccatttttcaaggccctgtagacttcttccacccttttaggctgaggctctttggggggattgttgtttttgtggcctaaattgtgcattttcttcagtttggcctgaggcttcttgagagcggaggaattttcaatgaaggagttacacctggatcgcctttcctggaggccgctgaaacccgcaaaggactggcttctaatgatcccattgggccctccaggcgaaaaagactgggatcctaccaacatgatttccgggagtctggtcggtagtcggttgagctggcgcctccggatcctgtccctccatggcctgtttctgatccagtgtaatcgcgaaggtaacaccatggtcccaacagagcggcctaaaacctgctcatggcaaaggaacaaaagggtcttgcagctatcctggaagttaagtccagacgtataaaaatgaaaaagaaaacttaacccccccctttttgttcttttcttaaaaaaaaaaaaaagagtatttgaggcttccgttgacttcttttatcttgtaacttgccttgcctttccttcccttaacttccgactggcccgaaggcagctgctgtgctgggctgccctagcctcctgtgccatgttttatgcatgaagatgatggggcggtaatttattcaagcagagacgatcaccgggctcctgtgtctgccctcgcgtcagaggagccg

SEQ ID NO: 11145 - RNA, 3764 nt, Homo sapiens
  source 1..3764: mol_type = other RNA
ctgaatagctgggactacaggtgcatgccaccacgcctgactaattaaactattttttttgtagagacagggccttgctatgttgcccaggttggtcttgaacctcctgggcttaagcaattctcctgcgttggcctcccaaagtactgggattacaggcatgagccactgcacctggcctacatttttatttcagttgtcgtgtctctcaggctctaaacaatttccagcccaaaccacagcaccatcctgatgaaaagggccagatattaagacagctgttaggcagttaacctgtaattaaaaggctgtggcaacttcagttccatgacgacctccgactttaacacagtctcgaggaaatttgtccaattgttcatatgccagccgcccatcttctcccagagacaagagggtttctgaggccacatttctgatttcttcagtatcagattgacacaatgtcaccagcattttaatgctttcagtagcctcaaggattttcagagccaggcaagctgctttctggagctggaggtttgtctttgttagtgcttcacagtaatagagcaaggccttttccctgaaatgctgatttttggaggctgctgccaagtaaagcgtcacagcctcactaacttcgttgtcctctctggttaatagcagagccagagtcctgagtacttcctgctgggccaggaggttgctgggagcaaggtcactcatggtttgtagcagtttttcatctcttagtgattgcagagtctgaaccatggaaacttgcctggccagctggctcaggtaactctccaggtcactgacgccgtggctggtgaagtaactgtaatactggaaaacagtgacgacttccgaggacaggctggaggaaagcagaggctcagcccggtccagaatttgggacaccagggttcgaaacactgggtctgcaagtcctggatattctttgttgacagttctggcaaagctggcctccagctgcttcatcactctgtccgctgggctgtggtagacaccaacagggctgcagcacttggtccagaatgacagcaaagacagctttttgtgaaattctggtatggcttccacaacagaactgatatttcctatgttctcatcactgacagctgcgagtttctccatcacttggatctgcctagaaagcttctctaagagacttcttgccacaaatggggttttgcttgagaaaacaatttgctgcacgagttgggtgcagtactggaggtgcctgacgatggtgatgtccaggctctcgttgcctgtggtcagtgggagaggacttcctgccacactggtcccaactcctgtgtcttcagtgagcgcttcactgagatgccccctggcttctgggtgaaccgacctgtaactgtgtttctcagtctcagtgtctgaaaatactgagtcagcacctccgccaacattacaaacctcatcaccatcctcctcctcgtcaaaatcagaggtgttcaggaaatcaaagctttctaaagcactttcaactgtgagacttaaactggaagacctgctgcggcttactgctggcttgcattttagaatatcatccaaattcatgacttcttggttcagatcctgaaactctttatactgctctttatgtggttctaatgcaagtaaaagcccattaaaagcatcctctaagcttccatctagaaaggatctgcagccttcagattctccaccaacagaaccctcagagagcagcctgtctgtggccattggcacctctgcagatgtgagcctcttgaccagctgctttgtgatgtttccttccgaagtgtccagttccacaggcttgagctcagaggcctcctcagactcttgcagaagtgcttctgcaacatcattctcaaggaacaggtgctcagccccagcacctgaggactgtcggcggcaagcctcagatggggccgaggcaggttttctgggctcctctgggtcttcctccttcaggtgtgactttggctcttggccttctcccagggagttcctggaagatgctgagctggtgtcatccataccctcattctgggaggccaagctgctgaggttaaactccgcaggggtgatggtaatttctggatttgttgagttggaaggggagcctgttgagtgggaggtgagggcgcagtccccgttgggcaggtcactgaagctgagcgacagtggcattttctcctcggctgcctttccattttcaaagatgtcatcaggtagatttgaatagagctctagcacggccttgggactcggcctgagggagggcaggtcactgaaggagcggctgcggtgcagcttggcaaagaaagtgtcttgcaaggcactcaagacagacagccgcctgggcttgtctggggaaggatgcagccacctaaagaaggagtggtctttgaaggtgggcgtttccggggtaccctggctgtacatggacattctcctctgaagggctgctgccttgttcccagcgcctgaggatgcggtcatgtcctccacgtcaaatggataccaggtgatttccaggttcagtttgatggtaccaaggtcattgatgtcgacagccactacctgaggtcgggctgcaaacagctctttggtctcacaggtcacgctacctaccaggatgtgagttgctagccctttgagctccgtgaccttgatggagatgaacccaactatcaggggcagaaaaactgtttcttctccatcccagctctgcttgccatttacttctattttgcctttcagtttccaccgctgccggccatacttcatgaaaatttcatattgatctccaggacagaggcgtgcaaagccagccagacctttcatcttgatggagaattctcccagcagattctctagctccacttcaatggtgcacatattctctgtgtactccttgaagctccgattgatctctgtcagactctcccgggcagctttgctggcaggggatgttgcgaaggcttgcttcattttgctggcaccatcctggaggcgtcgctggatacaataagcttcatagagttcatctaccttacttatatgaaactccaggcgtctcatgtatctttcaattgttttaatttgcttgtctaggtcatacagtacacccaggcgagagtttcttttcatatcttttaactgagctgtcaacttgtccagctccgtctggtgaacctccagatattcatcaagtccatttttcaaggccctgtagacttcttccacccttttaggctgaggctctttggggggattgttgtttttgtggcctaaattgtgcattttcttcagtttggcctgaggcttcttgagagcggaggaattttcaatgaaggagttacacctggatcgcctttcctggaggccgctgaaacccgcaaaggactggcttctaatgatcccattgggccctccaggcgaaaaagactgggatcctaccaacatgatttccgggagtctggtcggtagtcctaacgacgacggctccttgtcatgtcaggggcacactcagggttctctggcatataaaagcctccgcaccaatgcaatgcccggagctgcccgcacctccggctttgcagacagcctgagctggctcacttgggtgaaggggaccccgggaggaagtcgggtggacgcgagctgtccccagcgccggctgccctgccgcgtccgctcgcagcagctgcggcgcgcggggt

SEQ ID NO: 11146 - RNA, 3965 nt, Homo sapiens
  source 1..3965: mol_type = other RNA
ctgaatagctgggactacaggtgcatgccaccacgcctgactaattaaactattttttttgtagagacagggccttgctatgttgcccaggttggtcttgaacctcctgggcttaagcaattctcctgcgttggcctcccaaagtactgggattacaggcatgagccactgcacctggcctacatttttatttcagttgtcgtgtctctcaggctctaaacaatttccagcccaaaccacagcaccatcctgatgaaaagggccagatattaagacagctgttaggcagttaacctgtaattaaaaggctgtggcaacttcagttccatgacgacctccgactttaacacagtctcgaggaaatttgtccaattgttcatatgccagccgcccatcttctcccagagacaagagggtttctgaggccacatttctgatttcttcagtatcagattgacacaatgtcaccagcattttaatgctttcagtagcctcaaggattttcagagccaggcaagctgctttctggagctggaggtttgtctttgttagtgcttcacagtaatagagcaaggccttttccctgaaatgctgatttttggaggctgctgccaagtaaagcgtcacagcctcactaacttcgttgtcctctctggttaatagcagagccagagtcctgagtacttcctgctgggccaggaggttgctgggagcaaggtcactcatggtttgtagcagtttttcatctcttagtgattgcagagtctgaaccatggaaacttgcctggccagctggctcaggtaactctccaggtcactgacgccgtggctggtgaagtaactgtaatactggaaaacagtgacgacttccgaggacaggctggaggaaagcagaggctcagcccggtccagaatttgggacaccagggttcgaaacactgggtctgcaagtcctggatattctttgttgacagttctggcaaagctggcctccagctgcttcatcactctgtccgctgggctgtggtagacaccaacagggctgcagcacttggtccagaatgacagcaaagacagctttttgtgaaattctggtatggcttccacaacagaactgatatttcctatgttctcatcactgacagctgcgagtttctccatcacttggatctgcctagaaagcttctctaagagacttcttgccacaaatggggttttgcttgagaaaacaatttgctgcacgagttgggtgcagtactggaggtgcctgacgatggtgatgtccaggctctcgttgcctgtggtcagtgggagaggacttcctgccacactggtcccaactcctgtgtcttcagtgagcgcttcactgagatgccccctggcttctgggtgaaccgacctgtaactgtgtttctcagtctcagtgtctgaaaatactgagtcagcacctccgccaacattacaaacctcatcaccatcctcctcctcgtcaaaatcagaggtgttcaggaaatcaaagctttctaaagcactttcaactgtgagacttaaactggaagacctgctgcggcttactgctggcttgcattttagaatatcatccaaattcatgacttcttggttcagatcctgaaactctttatactgctctttatgtggttctaatgcaagtaaaagcccattaaaagcatcctctaagcttccatctagaaaggatctgcagccttcagattctccaccaacagaaccctcagagagcagcctgtctgtggccattggcacctctgcagatgtgagcctcttgaccagctgctttgtgatgtttccttccgaagtgtccagttccacaggcttgagctcagaggcctcctcagactcttgcagaagtgcttctgcaacatcattctcaaggaacaggtgctcagccccagcacctgaggactgtcggcggcaagcctcagatggggccgaggcaggttttctgggctcctctgggtcttcctccttcaggtgtgactttggctcttggccttctcccagggagttcctggaagatgctgagctggtgtcatccataccctcattctgggaggccaagctgctgaggttaaactccgcaggggtgatggtaatttctggatttgttgagttggaaggggagcctgttgagtgggaggtgagggcgcagtccccgttgggcaggtcactgaagctgagcgacagtggcattttctcctcggctgcctttccattttcaaagatgtcatcaggtagatttgaatagagctctagcacggccttgggactcggcctgagggagggcaggtcactgaaggagcggctgcggtgcagcttggcaaagaaagtgtcttgcaaggcactcaagacagacagccgcctgggcttgtctggggaaggatgcagccacctaaagaaggagtggtctttgaaggtgggcgtttccggggtaccctggctgtacatggacattctcctctgaagggctgctgccttgttcccagcgcctgaggatgcggtcatgtcctccacgtcaaatggataccaggtgatttccaggttcagtttgatggtaccaaggtcattgatgtcgacagccactacctgaggtcgggctgcaaacagctctttggtctcacaggtcacgctacctaccaggatgtgagttgctagccctttgagctccgtgaccttgatggagatgaacccaactatcaggggcagaaaaactgtttcttctccatcccagctctgcttgccatttacttctattttgcctttcagtttccaccgctgccggccatacttcatgaaaatttcatattgatctccaggacagaggcgtgcaaagccagccagacctttcatcttgatggagaattctcccagcagattctctagctccacttcaatggtgcacatattctctgtgtactccttgaagctccgattgatctctgtcagactctcccgggcagctttgctggcaggggatgttgcgaaggcttgcttcattttgctggcaccatcctggaggcgtcgctggatacaataagcttcatagagttcatctaccttacttatatgaaactccaggcgtctcatgtatctttcaattgttttaatttgcttgtctaggtcatacagtacacccaggcgagagtttcttttcatatcttttaactgagctgtcaacttgtccagctccgtctggtgaacctccagatattcatcaagtccatttttcaaggccctgtagacttcttccacccttttaggctgaggctctttggggggattgttgtttttgtggcctaaattgtgcattttcttcagtttggcctgaggcttcttgagagcggaggaattttcaatgaaggagttacacctggatcgcctttcctggaggccgctgaaacccgcaaaggactggcttctaatgatcccattgggccctccaggcgaaaaagactgggatcctaccaacatgatttccgggagtctggtcggtagtcggttgagctggcgcctccggatcctgtccctccatggcctgtttctgatccagtgtaatcgcgaaggtaacaccatggtcccaacagagcggcctaaaacctgctcatggcaaaggaacaaaagggtcttgcagctatcctggaagttaagtccagacgtataaaaatgaaaaagaaaacttaacccccccctttttgttcttttcttaaaaaaaaaaaaaagagtatttgaggcttccgttgacttcttttatcttgtaacttgccttgcctttccttcccttaacttccgactggcccgaaggcagctgctgtgctgggctgccctagcctcctgtgccatgttttatgcatgaagatgatggggcggtaatttattcaagcagagacgatcaccgggctcctgtgtctgccctcgcgtcagaggagccg

SEQ ID NO: 11147 - RNA, 3633 nt, Homo sapiens
  source 1..3633: mol_type = other RNA
ctgaatagctgggactacaggtgcatgccaccacgcctgactaattaaactattttttttgtagagacagggccttgctatgttgcccaggttggtcttgaacctcctgggcttaagcaattctcctgcgttggcctcccaaagtactgggattacaggcatgagccactgcacctggcctacatttttatttcagttgtcgtgtctctcaggctctaaacaatttccagcccaaaccacagcaccatcctgatgaaaagggccagatattaagacagctgttaggcagttaacctgtaattaaaaggctgtggcaacttcagttccatgacgacctccgactttaacacagtctcgaggaaatttgtccaattgttcatatgccagccgcccatcttctcccagagacaagagggtttctgaggccacatttctgatttcttcagtatcagattgacacaatgtcaccagcattttaatgctttcagtagcctcaaggattttcagagccaggcaagctgctttctggagctggaggtttgtctttgttagtgcttcacagtaatagagcaaggccttttccctgaaatgctgatttttggaggctgctgccaagtaaagcgtcacagcctcactaacttcgttgtcctctctggttaatagcagagccagagtcctgagtacttcctgctgggccaggaggttgctgggagcaaggtcactcatggtttgtagcagtttttcatctcttagtgattgcagagtctgaaccatggaaacttgcctggccagctggctcaggtaactctccaggtcactgacgccgtggctggtgaagtaactgtaatactggaaaacagtgacgacttccgaggacaggctggaggaaagcagaggctcagcccggtccagaatttgggacaccagggttcgaaacactgggtctgcaagtcctggatattctttgttgacagttctggcaaagctggcctccagctgcttcatcactctgtccgctgggctgtggtagacaccaacagggctgcagcacttggtccagaatgacagcaaagacagctttttgtgaaattctggtatggcttccacaacagaactgatatttcctatgttctcatcactgacagctgcgagtttctccatcacttggatctgcctagaaagcttctctaagagacttcttgccacaaatggggttttgcttgagaaaacaatttgctgcacgagttgggtgcagtactggaggtgcctgacgatggtgatgtccaggctctcgttgcctgtggtcagtgggagaggacttcctgccacactggtcccaactcctgtgtcttcagtgagcgcttcactgagatgccccctggcttctgggtgaaccgacctgtaattttagaatatcatccaaattcatgacttcttggttcagatcctgaaactctttatactgctctttatgtggttctaatgcaagtaaaagcccattaaaagcatcctctaagcttccatctagaaaggatctgcagccttcagattctccaccaacagaaccctcagagagcagcctgtctgtggccattggcacctctgcagatgtgagcctcttgaccagctgctttgtgatgtttccttccgaagtgtccagttccacaggcttgagctcagaggcctcctcagactcttgcagaagtgcttctgcaacatcattctcaaggaacaggtgctcagccccagcacctgaggactgtcggcggcaagcctcagatggggccgaggcaggttttctgggctcctctgggtcttcctccttcaggtgtgactttggctcttggccttctcccagggagttcctggaagatgctgagctggtgtcatccataccctcattctgggaggccaagctgctgaggttaaactccgcaggggtgatggtaatttctggatttgttgagttggaaggggagcctgttgagtgggaggtgagggcgcagtccccgttgggcaggtcactgaagctgagcgacagtggcattttctcctcggctgcctttccattttcaaagatgtcatcaggtagatttgaaaagaaggagtggtctttgaaggtgggcgtttccggggtaccctggctgtacatggacattctcctctgaagggctgctgccttgttcccagcgcctgaggatgcggtcatgtcctccacgtcaaatggataccaggtgatttccaggttcagtttgatggtaccaaggtcattgatgtcgacagccactacctgaggtcgggctgcaaacagctctttggtctcacaggtcacgctacctaccaggatgtgagttgctagccctttgagctccgtgaccttgatggagatgaacccaactatcaggggcagaaaaactgtttcttctccatcccagctctgcttgccatttacttctattttgcctttcagtttccaccgctgccggccatacttcatgaaaatttcatattgatctccaggacagaggcgtgcaaagccagccagacctttcatcttgatggagaattctcccagcagattctctagctccacttcaatggtgcacatattctctgtgtactccttgaagctccgattgatctctgtcagactctcccgggcagctttgctggcaggggatgttgcgaaggcttgcttcattttgctggcaccatcctggaggcgtcgctggatacaataagcttcatagagttcatctaccttacttatatgaaactccaggcgtctcatgtatctttcaattgttttaatttgcttgtctaggtcatacagtacacccaggcgagagtttcttttcatatcttttaactgagctgtcaacttgtccagctccgtctggtgaacctccagatattcatcaagtccatttttcaaggccctgtagacttcttccacccttttaggctgaggctctttggggggattgttgtttttgtggcctaaattgtgcattttcttcagtttggcctgaggcttcttgagagcggaggaattttcaatgaaggagttacacctggatcgcctttcctggaggccgctgaaacccgcaaaggactggcttctaatgatcccattgggccctccaggcgaaaaagactgggatcctaccaacatgatttccgggagtctggtcggtagtcggttgagctggcgcctccggatcctgtccctccatggcctgtttctgatccagtgtaatcgcgaaggtaacaccatggtcccaacagagcggcctaaaacctgctcatggcaaaggaacaaaagggtcttgcagctatcctggaagttaagtccagacgtataaaaatgaaaaagaaaacttaacccccccctttttgttcttttcttaaaaaaaaaaaaaagagtatttgaggcttccgttgacttcttttatcttgtaacttgccttgcctttccttcccttaacttccgactggcccgaaggcagctgctgtgctgggctgccctagcctcctgtgccatgttttatgcatgaagatgatggggcggtaatttattcaagcagagacgatcaccgggctcctgtgtctgccctcgcgtcagaggagccg

SEQ ID NO: 11148 - RNA, 2814 nt, Homo sapiens
  source 1..2814: mol_type = other RNA
ctgaatagctgggactacaggtgcatgccaccaggcctggctaatttttgtattttttgtagagatgaggcttcaccatgttggccaggctgctctcgaactcctgtgttcaaacaaatccacccaccttggattcccaaagtgctgggattacaggcaaaagccatagtgcccggccctgattttaagtttttatctgaaaagtacccctaacacacacttacatacaaagtgaaaatcaattccaccactaaaaacatttacaatacggaaggcagaatagccctgcaaacttcctccctctacctcacctgccccccacaccccccaatcccactgctcagaggaaacctcggtgatttttcccagcaatgctgattcagacatcatttgcctctgatccaaactgaaacatagggctctgggcacaggcatctcccagaagcttctccggtatttcttagaatccgtgtactgtctcgccttacctgcccttcagctctggtcatgaagccaaggagggcaggtcttcttcacttgtagtgctactctgaaggcacaaatacaacctgcggggttgaggcggatgctggaggagggcatggggctgccgagggaagcacttgttaccagtttaatgccggggttgcagggctagaggagacaggattccactgtgtttggagatgaagttcccactccaaatgcagacaggggaagctagcaatttcagttctcagcattgaaaaagttttggccatgaaagtagaaatcacagctcaagggagagatttcctgattcaagataaaatgctcagacagtcaacaaatcatgcgggaagaggctctatgtaaaatgttacgtttaaaaaaagattcaacatacctgcccatgtaccccctgtatctaaaataaaagttgaaaaatttttaaaaacttacaaaattgtgcataaatctcaaatggatgaagtcaatttctatatgtctatctctttatgaatattcagacataaacagaagaaacccaaattgaaatatataaaaatgttactaaagttgtactttatttttacctgtatttttccatttttctttaatgagaatggatttctcttgtagtaaaatgttatattgaaacaaagattgaatgctacatctatagtaacttaaactgggttttgaaaaaaagggactaaatgtagggttacaaaagatatgtgaaaaccagcaccagacactgggaggaagaatctcttttgagcctcagtttctcagtaaggagatgcttaaatagttccatagagttctaagtgattcacaatccctgaatcaactctgacaagtgaagcttgggctggggttttaaaaattatatcccctactttgtcctgtgtgagaaggaacttgtgcaagcagtttcatggtccccagtggtctttgaagttctggggtgcaggagggtttgaggctgcctggggcgatggttaggactgctctcagagcaggtgaagccgcaggtctctgagcgatcctgaaagccctgctccttcagcacaggtgccccgggtccagagttttctgttagggaatctggttttctccccgtaggtgtgaggccttcttaccatgacctcccatttgacgtcattagatcaatatctgcatttccccctctctgttactctatagttaagaatatatactacacattggtgcgtaagagtggaaagtaaaaatatcatttcgacatgactgattttcacactgaacatagtgaaaaccctctttaactctatggggctgtgttctactccagagggaccagggaaccatctcacattctgctgaggactcttttgcgccctcctcagacgatattaatgcaaaagaaggcaggtcattttcttgttttagatgagagaaattgaagatttgattttggctaattttataatagcaatttaaaatatttattccctcaggagtcagaaataaatctgtaggaatagcaaggtttccaaatattaacatttgcttttggttcagactttcaaaagcctttattcccactcttcccccaacctctctttaatttcacctgttctgagcactttgagtactaaacaatggaatctcagatgcttctggcaactatgtgttattagtcaggaatggcaccttgttatttgattgcattttattgtttccttcagctcaatgtgtacctgatattggagggctctccctatgggttgagattgagacatgttataaatgatgtggtttttattatttctgtgggctcctgtgcagccaggtgacaatcctgaggctgcgtaagctggaggtcaggcccgagttgccctgttctgactagcagagcccagtgtccacaccgtggcacagccacttctgcctgcatcatagaatggctggggcagctgctgttgtgccgacttgagatgcctgttccatgaggagatcagtaggcattcagcacggctatcctggccttttcacacagtgggtctagtttaccatcgcctccgaactccaagtccttaatgttgcagtggaagatgacttcttcattcaccatgagttccaccacattccagtcttctatcttctctaggatgacctcatgtccatctatggccaacacagcttgcaggccctgcaggcggaaggtgtggtgctccaccggtaggcctgccgcgctgtagggcccatagcgcaggatgaccactgcgttcttgggcatcgccaggcctccgccgccgcagaggcaagggagaaacacacgctgct

SEQ ID NO: 11149 - RNA, 1879 nt, Homo sapiens
  source 1..1879: mol_type = other RNA
ctgaatagctgggactacaggtgcatgccaccatacccagctaatttttttattttttgtagagacagtgtttcgctatgttgcccaggctggtcttgaactcctgaactcaaacaatccatctgccctggactcccaaagtcccaaagagccaccatgcaagtcctaagaactggttgtaattttgttgtagccaatgcttcccaagaaattcctgggggtgaaatggttaacagttttattccctcctcttctcactatctccactgtcactccccagctcagaccaacctcatctctcactgtccactgtcatggcctccaaatctggtctctccattcacctcctgcttattttgcatcctttttcctcttaacacagagtgatctctttagaatataaactggctttccactgcattaaggtaaaatccaaacttcttcccatgatctataaggtcccataccatctgacgctgggcccacaccatctgacattgggcccacatctccaactttgactattattttcttcctcattaactgcaagtctcactggcctcctcccagctctttcctgttcctggagatttgctgtcgcatctgcctagtgtttctgagactttttacagctcttaatccttcaggtgtcagcttaactatcttatcgtcaggcaaagatttgttgttacttttttttttttttgagacagtctctcactctgcctctcactgaggctgaggctgaattgctcactttaacctctgcttctcaggttcaagtgattctcctgcctcagcctcccaagtaggtgggaaagcaggtatgtgccaccatgcctggctaatttttgtatttttagtagaggcagggttttgccatgttggccaggctggtcttgaactcctggcctcaagcaatctgcctgccacagcctcccaaagtgctgggattacaggccaggcaaagcttttgtaaccacctaaagcacagccttctcccttgcccttctcgatgttactccctatcacagtagttttcaaaatgtggtcctgaaaccaacagcatcaggaacatctgggaacttgttaggaatgcaagttctcaggccccaccctagacctgctgaatcagaaactctggggtgtggcaaatccatgtgtattagcgagcccttcaggtgattctgatacaggctaaagtttgcgcagttctatggcagtatcctgtttatttcctacatgtttatcgtaaactataatcgtttcttcttattatttaatgcatttagcttttctcactagatttgcaagcactgtaaggatcagcaatcattgttgaggtacaagacaatatctgaggctgattaatatttgctgaatgaatgaatgacacggaacatatcttggaaaatactgctttacataggatctatattagcttatggctaaacttcaattgccgtgaaccaccttaccaatatttctttccattcatttattcaacatttattgacatttgtaatatgctaggcactatcccaaatgctataaatacaaacacgagcaagtccttgttctgaaagaacttatagacaagtgagataaaaacaggtaaatacacaattattttattctgataagtgttattataaggcctagaaaaacctaccaaaagcattaaaaatacacatgtacttgtctttgacctagttattctagttctaaaaattaattctaaaaaaaacccagggatgcatacacagatttatcaaaacgatgtttgtcagcattatttatactagcaaaaaaaatcagaaataacctaaatgtaaaagaatggagaatttggctgggtgtagtggctcatgcctgtaat

SEQ ID NO: 11150 - RNA, 1999 nt, Homo sapiens
  source 1..1999: mol_type = other RNA
ctgaatagctgggactacaggtgcatgccaccatgcccaactaatttttttgtatttttagtagagacggggtatcaccatgttggccaggatggtcttgatctcctgacctcatgatccacccgccttggcctcccaaagtgctgggattacaggggtgagccaccatgcccggcccagaaataatgagatttttcaaagcaacagtgattcatcacactgaaataggactctacagttcaaaatgacaagaataactttatcctgtgttacataccaatattagagaaatcttaaaagtttgtagctgttagtttttagtttatgcatgtagttcagtagcccaagttgacaactcccctgtctctctacatgaatcactgtagttgaaattgtactaaagtatcagaagtaacatttactgtaaaatgttaaatagcaccaatattacttgaaagtaaagtgagacattaataggaatgctgacacagatttaatttctaactactagagagaaagcatctcctagacaaaatactatttagatatgaattattttaagatcacagccagaaaaatgtcataaaacattttagattttgcttggaaaagttagaaaagaaagctttgtgtatcgctcttttatcttttatttccaaagaagatgtacaaatgcttacataatcagaacagtgcaatcttaccaatgaagtttaccttgtgggagctacatttacttatttcatatattagttcaacaacataaatataataaaaatgcttttaagcaatctgattagagcaacatttatattaactacaaaatatacagtaaaatgaaacatcttgttaaataggcctgtaggaaaacaatattttaaaggaatacattttcatgaatctactttcatatttatttgttttattgtatcttatagttactataatcgttgtgtgcttttgttactgcaatttccaggatcattgtatattctcagtatgccagtgactatatatgtaaaggtaatttaaaaagtattactcccagagtaaaaacagacaaacaaataagaaatctcatttttaatgggaagttgtgcataaaactattgtagtatttttatagaaatgtcccttaatcattataagttcatcattataaaatgtatactattgtactaaagcaaaactgtctgcctttaaatctaagtggtgtcaacttactgtataattctggttacaaagttagatatgaaatctttggctattaattagaaaagcattatttgaaaagacctgtcaataaacatttctaaatgtggttgctcatcttaatagttttcttaattagaacagctaggaaatgaacagaacagtggtgcttttatgttataataacaaagaagtattacagtatcccaatctccagacctggggtccaagtattcaatcctggctcagttgcaggctgacagaagagaagcatcgtcctacgctcgtacacaatggagcaatgataacatctgtcacactcttccatattgtctgcactgaaggcagaaccattaggcaggtctttacaaaaggcattaaaatccagatgtgcagacagctgagggtggcaaagagaattcccgcaatgaaggccaggggaatggccaggaacaccgtcaggaacttgtacattacgtatttgctgatttcaaagagggcatggctgcagatccacactttgtcaaaggagtgcgtagtcaccggctctgcgatcacatcctcgaagcccagctgaggagacaggacgcagggaccccgaactgtcagccaacctgacgccccgggaaccgggagcgctttgggcgggggaagcaggagggaaggacgtgccagggcgtccgcctcttctcttagggtcacggtgggcgcacaggaacctggctaagaattcctggctacgcgggcggcctggtgacgggtgggaccggggaagggtgcgggtctc

SEQ ID NO: 11151 - RNA, 1979 nt, Homo sapiens
  source 1..1979: mol_type = other RNA
ctgaatagctgggactacaggtgcatgccaccatgcccaactaatttttttgtatttttagtagagacggggtatcaccatgttggccaggatggtcttgatctcctgacctcatgatccacccgccttggcctcccaaagtgctgggattacaggggtgagccaccatgcccggcccagaaataatgagatttttcaaagcaacagtgattcatcacactgaaataggactctacagttcaaaatgacaagaataactttatcctgtgttacataccaatattagagaaatcttaaaagtttgtagctgttagtttttagtttatgcatgtagttcagtagcccaagttgacaactcccctgtctctctacatgaatcactgtagttgaaattgtactaaagtatcagaagtaacatttactgtaaaatgttaaatagcaccaatattacttgaaagtaaagtgagacattaataggaatgctgacacagatttaatttctaactactagagagaaagcatctcctagacaaaatactatttagatatgaattattttaagatcacagccagaaaaatgtcataaaacattttagattttgcttggaaaagttagaaaagaaagctttgtgtatcgctcttttatcttttatttccaaagaagatgtacaaatgcttacataatcagaacagtgcaatcttaccaatgaagtttaccttgtgggagctacatttacttatttcatatattagttcaacaacataaatataataaaaatgcttttaagcaatctgattagagcaacatttatattaactacaaaatatacagtaaaatgaaacatcttgttaaataggcctgtaggaaaacaatattttaaaggaatacattttcatgaatctactttcatatttatttgttttattgtatcttatagttactataatcgttgtgtgcttttgttactgcaatttccaggatcattgtatattctcagtatgccagtgactatatatgtaaaggtaatttaaaaagtattactcccagagtaaaaacagacaaacaaataagaaatctcatttttaatgggaagttgtgcataaaactattgtagtatttttatagaaatgtcccttaatcattataagttcatcattataaaatgtatactattgtactaaagcaaaactgtctgcctttaaatctaagtggtgtcaacttactgtataattctggttacaaagttagatatgaaatctttggctattaattagaaaagcattatttgaaaagacctgtcaataaacatttctaaatgtggttgctcatcttaatagttttcttaattagaacagctaggaaatgaacagaacagtggtgcttttatgttataataacaaagaagtattacagtatcccaatctccagacctggggtccaagtattcaatcctggctcagttgcaggctgacagaagagaagcatcgtcctacgctcgtacacaatggagcaatgataacatctgtcacactcttccatattgtctgcactgaaggcagaaccattaggcaggtctttacaaaaggcattaaaatccagatgtgcagacagctgagggtggcaaagagaattcccgcaatgaaggccaggggaatggccaggaacaccgtcaggaacttgtacattacgtatttgctgatttcaaagagggcatggctgcagatccacactttgtcaaaggagtgcgtagtcaccggctctgcgatcacatcctcgaagcccagcttgagatgcgagttgagccggtggggatcccggtcctggtccgagtccgcgaacttctcggggtcggcgtactcgaggccgctgtggtggctgtaggagtcgtcgtccatgaagagctgtacgtccgccttctccgtctccagccccatcgcagccttggtgcgcggccgctgcagcccggctggcgcggtgc

SEQ ID NO: 11152 - RNA, 1791 nt, Homo sapiens
  source 1..1791: mol_type = other RNA
ctgaatagctgggactacaggtgcatgccaccatgcccaactaatttttttgtatttttagtagagacggggtatcaccatgttggccaggatggtcttgatctcctgacctcatgatccacccgccttggcctcccaaagtgctgggattacaggggtgagccaccatgcccggcccagaaataatgagatttttcaaagcaacagtgattcatcacactgaaataggactctacagttcaaaatgacaagaataactttatcctgtgttacataccaatattagagaaatcttaaaagtttgtagctgttagtttttagtttatgcatgtagttcagtagcccaagttgacaactcccctgtctctctacatgaatcactgtagttgaaattgtactaaagtatcagaagtaacatttactgtaaaatgttaaatagcaccaatattacttgaaagtaaagtgagacattaataggaatgctgacacagatttaatttctaactactagagagaaagcatctcctagacaaaatactatttagatatgaattattttaagatcacagccagaaaaatgtcataaaacattttagattttgcttggaaaagttagaaaagaaagctttgtgtatcgctcttttatcttttatttccaaagaagatgtacaaatgcttacataatcagaacagtgcaatcttaccaatgaagtttaccttgtgggagctacatttacttatttcatatattagttcaacaacataaatataataaaaatgcttttaagcaatctgattagagcaacatttatattaactacaaaatatacagtaaaatgaaacatcttgttaaataggcctgtaggaaaacaatattttaaaggaatacattttcatgaatctactttcatatttatttgttttattgtatcttatagttactataatcgttgtgtgcttttgttactgcaatttccaggatcattgtatattctcagtatgccagtgactatatatgtaaaggtaatttaaaaagtattactcccagagtaaaaacagacaaacaaataagaaatctcatttttaatgggaagttgtgcataaaactattgtagtatttttatagaaatgtcccttaatcattataagttcatcattataaaatgtatactattgtactaaagcaaaactgtctgcctttaaatctaagtggtgtcaacttactgtataattctggttacaaagttagatatgaaatctttggctattaattagaaaagcattatttgaaaagacctgtcaataaacatttctaaatgtggttgctcatcttaatagttttcttaattagaacagctaggaaatgaacagaacagtggtgcttttatgttataataacaaagaagtattacagtatcccaatctccagacctggggtccaagtattcaatcctggctcagttgcaggctgacagaagagaagcatcgtcctacgctcgtacacaatggagcaatgataacatctgtcacactcttccatattgtctgcactgaaggcagaaccattaggcaggtctttacaaaaggcattaaaatccttgagatgcgagttgagccggtggggatcccggtcctggtccgagtccgcgaacttctcggggtcggcgtactcgaggccgctgtggtggctgtaggagtcgtcgtccatgaagagctgtacgtccgccttctccgtctccagccccatcgcagccttggtgcgcggccgctgcagcccggctggcgcggtgc

SEQ ID NO: 11153 - RNA, 3906 nt, Homo sapiens
  source 1..3906: mol_type = other RNA
ctgaatagctgggactacaggtgcatgccaccatgcccagctaatttttgtatttttagtagagacagggtttcaccatgttggccaggatggtcttgatctcttgacctcgtaatccatctgcctcagcctcccaaagtgctgggattacaggcgtgagccaccatgcccggccggctttcactttctctgaggaatgcagctctttctgctactgactgcctcgggtagtcttcccaccccatcttctatgccaattttagccccttatacccaaatcctagcacgcagatggatgagggtgggtgcaactgctttgaatgggtcatttgaaaaaaacagatgtttttcagtcttcttgtacaaatttttctttttgcctgtttcttagcatagcacaacagagaacatggaaataagtcattttcatgctattagcacatttaggaaacaggcttctacagtaattaaactaatgaagatgaccctagattcaagaaacagaaattagagttgactgaacaggcattaggggaaatgaagacattcacattcaaaaaaagatgagattttaaaataagaaatcaaattaataatagcccaaactctatcaagcaggaaagagcttctaatgactcaaagaagacttggagacatatgtagattagtctatcatattcaagtgaatataaaaatgatggtatcttatcataaaaataagaacattaagggacagactgaaggaaagcaaaaaagtagaagaaactggctaactatatacaacttaaaccaaaatggaaaggcttttctttgaaaaaaaactttttctccatgtaaatttttagttgttattttccaaacatcaacaaccagcttttaaagtagcaactcaaatccactgcagtaaataaatgcaattcagaaacaaacagaagctccattccagtggtgcaaggcccccatcactgcccatctggctcccttcagtaaataactgtgcggctctggtgtcaatcagggtgacggcatgatcagaggatttctatctgcagtttgagtagatctatctctggtaatcattagcaatgacaacagttattactggcttcttttcttttttctttttttttttttttagacagagtctcactctgtcacccaggctgaaatgcagtggcgcaatctcatctgactgcaacctccacctcccgggttcaagtgattctcatgcctcagcctcctgagtagctgggattacaggcatttgccaccaagcccagcttatttttgtatttttagtagagatggggtttcaccatgttatccaggctggtctcgaactcttgacctcaagtcatctgcccacctcggcctcccaaagtgctgggattacaggcatgagccactgcgcctggccccaactggcttattttctgtcaaactcagtgtttgatagaaacagtctagtatgtcaggttctctttttaaccttactgattccagaggccacaatggaggggaaaaggctagcataaggaagagtttcctcaaatgccttctctaggctacgatttttatgtaaaggctgattaagtggtttgctgggatctggagctgcccaaggaatttctgcccactcggaaggccactggtgtcctgagtgttgctcattcagcagaatgaagcgctctgtcaagctgtgaaggccactggtgggggaaagagggaatatgctcattcttgttattgctgttgctattaataaacagggctttatggattaaaaggggagagagctatgacattattaacattaattcttcttcattaactaatctttgaattttttaggtttttttttctctttaggacacataagcccagccaagattcaaaggcttccttttataaactaaagtacaatatttctgtgtcattattatatatagccttgagtaatcacaattaatgtgatttttaatgcacaaattaaacatgctataaactctaatgatgatcatgcaggattttgatcactatcatcattaggtgaaacctcagaaaaaaatgtaagcctatcatgggtcctaacagctttttattttaattctacagatttgggcatattggctgttgagagagagaaaaccaaaaccttctctttttccatctggctatgagtgcttttcatagcttattttttccacactcacccctaaaaaatgcactggagctgagctattgtaagaatgtgtcagattcaaatgattatatcattgactatctgctatttcacaggagaactgaactgtctgactttttaaaaaactcagcacggactttatagtagcgagactttatcaacagtgagttagtgttacaggtgacttggctcataaaaaattaaaagcttcagaaattaactttatcacagaaaacatttagtcataagcaacccccagttgtagaggcagagaaccaaagatcagagatatgtgccaaaaaatacttttcagaccccgagcaaagagaatagtaagagctggtgtcagcccattgcggtgccaggctgagctagctggtaaggtctctggtaaagaaaacgcttttctgggacgactataatgggcactctgtgagctccggggcctggagttgcttttcgacagatgactttgttccttctttacatggtaaagttcagtttatatttttgtagaaatacattcttgacatttccaatgaaaatgctgacttggtcgcattttagtttcattctaattggaagaaatgagccctcgcttgtttggaaaacaaaaggctacgaaaactcgtgttcattttgggaacttttattaagtattcaaaacagaatgaaagtgatctagttctggaaaagcagggtcatatctaaaattaaaaacaaaaactaggttgctgagagagatcaaaagacaaaaggaattcactaagcagatgaaagttaaaaacacggcatatataacctcatcacctgaggtacgctgatttaatatcagcagcgccaacaaaaaaagtaaaatcataatgggctcccatctctccaaaagcaaatcaatgcctcattgtgaaaagaaacccacaaagagatggtgattttacttttatttcaaagaccaaataaagtctttggtcctgtaagcaagttttaatactgtaacaagattgctaacttttgctgtcagtctgactcataaaggacttaattacttttttcgacagtcaagaagggtccactcagagaaattgtgtggcagagaaaaaagggcagcgtggccaagaggaacctgtaatgatgcactcgtcaattacagctatttctttcaaacttgtcttgttaaatttaccttcctttccagacgtcataaattagccctccattaaagcatctgaatgccaaacagtacattattcttcacaaggtgaccatcaggagcaggctatgctggaattgtattcttttccaattggctgctaatatcaccactcctggttcttcctttctttcttgattcaagagcctcttcccatcacctgaattgcttcaataaagacacagacttaatttgtggttcttcaataaattcaaagagaaagttacaacgtgcattgaagagacacattcttgttaaaaggcattgtgggaagccaccattcttggtggtggattccagcaccttgaaacaccacaaactggaagagcaagcaaggagccaatggctaattctaccacagacaactatgctcagcaagggtgagctaagggaattaaggatacaataaaataatggggccaagcatggtggctcacgcctgtaatcccagcactttgggaggccgaggtgggtggatcatgaggtcaagagc

SEQ ID NO: 11154 - RNA, 4632 nt, Homo sapiens
  source 1..4632: mol_type = other RNA
ctgaatagctgggactacaggtgcatgccaccatgcccagctaattttttgtattttagtagagacggggtttcaccgtgttagccaggatggtctcgatctcctgacctcatgatctgcccacgtcagcctcccaaagtgctggaattacaggtgtgagccaccgcacctgggcaagtgacctaatttttgtagagcatgccttcttacttgttttccatcataattaatatgatgcatttgtcagcggaaggtcttggaaatggggcaatgtgccatctggaaagttccctcctgcatgaaactggcctgagtaggtggataaatccattactttagggcattgttctcctatcagttagctgatgaggacaagtccactcatatgatgtggcagtgctgagtctttgaagaggttgcgtttttaataaacagttcaaaacaataaaccccaccccaccccacctaacttcatttgcctcttctttcggtgatctcaggaaccagagtcagagttgtactttttacccttaactcttcacagcacgtgagtgtgcaatcattaggctccatctcaacaatccttgagaacagagcacacctcatctttcaaatctcacctagtgctgggaacaacacaaagtcctacaaatgtgataatgaaacaaactgaccctgaatcccacaggctctgaacagatacattagggaagcctgagcctggagcctgctctccaactgagcagcaggagagatggggtggcacaggctttcaaaagatgcagtgggctgcagcaggcagacatttgggggagaagtgactggaaaaatacaaccatccagggggaagatgatgaagggactgggttcacacatggacagcaggcttcagaaggacgccagcagaatgaatgtggagtggatgtactcactctgcattgctccagaggacagggtaagaccccaggctggaagtcatgcagaagcagataaggcacacacaagctccgcacagggagaaacttcttagaaactcagcgggatgggtaacttcattagagaatgagatttcctcactggacattttcatctggaggctgcaggagcagtggtcaaagatgatacagacaggattcctgaatgccaaagttcctccctcgataggatttggaggctctcgggtgatggaccaacaccatcctgtgggcttgtggaggggaggatgacaacctgcataagcacagccatcactgagtgtaacttcaggctcgtgagccatcctcagtgcatcaactcagtgggggatgaggacggaggccagggatgggaagcaacaggaaaggaattgctggcctgtgcctttgctcagaatataaatattctggtagaaactcccctcaaggaatgtggtcacaagttaccctctgggcccctgagcataaacccacaccatcatgtacatgggaggagaggagcaccttctcatacccaggatcactgggcatagactcccttcctcactacaaacgggttggagagatccaaagatgctctctaaaaacaaagtaacaatgtgagaaaatggcaaaatagggacccgcagtaagttcaatcttcccagtgaacttcattaaaaatttcatctgattacaagtgattatacttcaaatacctacaggagcctcactggatgtgggtgcagcattcgttcctgaggcctcagaagtgctctcctgagcacagccagtgcaaatttgcagggtgagaagtcaaaggcagaaggaagcaggtgagagcattccctgcctctaaagaaaaagagctctccttattcaaaacatcaagttctactgaaccaagttgcagatcttaacaataatagagatcactgtaaaagagaaactttatgctaaaaattttttttaggaggtaacatcctggtgtttctcagatgcaggtaaatcatgaccttccacattctctttcaacacagggagcacctgagatcctacagacaggaaacatggggaggataaatccaatgatgcatgcatcaggtacatgccaaagttcacctttgtttcacgactctcagaaagtttttggaaaacatgctggtttcgttgcccagtttgctggtcgatgcaaatcatctggcatctgtgacaaggccccaaaacctggaaacgcaaagagccaattgaaatctcatcccatttctcttcttcaaaagccctttttccattgataataatattggcacgaaaacgcaagctgagatccttcagtgagaataattcctcctttccattctcatcactggtgtttagttgccggtgaagttccaaaatactggatgtgttgatcagcagatactgtgcctcattcaccagagaaagggtggccattgtaccaggaagttgatcttttccatgtttcttctttgcattcctttgagagtttgaactttgtttgatcaaatgacaaggacggccaaaaaatgttgacaaccagcttgaaattttttctccacaatcataagtacttactctgtcagcacagaccctgctttggcgaatctgagtccgttcactattttcctcaagaggcacctctataggctccatccctttggctttgatgaccatgatcctttgccgcaagtcgatgaagggctggatcaggcagagccggggttcctgcttctgactcaggcaaacaccattgtgattcacaaccatccagctccggtcatatagcagcccttggtttcctacaggccacctggtcacctcaaatgcagcacaggatttgattggatagagataaaggttagtgacaacatgtggcccaagggccccctccaggactcctgcagctttctctgaaggagtcggctgggttctggcgacatcacacacaggtggggccacaggcacagcattcacagtagacgagttgttccaaaccctggagcctgtgagggcatcttcctgaggcgagaggctacgtctgcccatgacagcaggtataacatcagcctggctgtctgctgatggggctccagtctccccggtgtcagcatgggcctgagggacaggccagtcccctgatgagtgcaggcgagtgtctatgatgaacctaagaaaggcctggacatcatccagcgtcgacatgtatccaaatgaaatcctcacagatcctgtgggctgcccatctatgaggtccatattgtccccacagacatgaccagcctgaaaatgcttcctgaccatctcgttgcttatgcccaggtgcctctggcaggccccagtgttacagaagcagccagttcgcaggtggatgttgtaaagactggccattttgtccacctgggagtaaccaatgatgttccctttgtcatccagcacattaaaattgatgattgggccctgaacctcagggctgctgaactcagaatcgctgtaaatccgcaccacaggggctccattggggtactggagagaggacagggccacgtaggtatactgagccaaggtgaaggtgtgctgctttatattctccattccacctgtgaggcgctctagggtgtcaaatccatgttttagcgcgataacatcaaggaatgagatggtgccatcttcaaacctctgagctaccgactgcctcgggatgtagaagtcttctcctgctaggtacgcagaggctgtccctcctccaaagtaggtcttcctcagtagaggagccgcacgattatggaccagcagagcgcccaggcctgtaggaaacccgaagatcttatagaaggagatggggacaaagtcggcctggtgagctgacaggtccaaaggcgaggtgctcacgtaggaggctgcatccagcagcacaaaccacttcccaggcgtgctcacagggtgcaaccgcccagacttgacctcttctatccaggacagggggtatctgactccagaaaagttactctgagctgggtagcagaagagatgcggcagctggcagtctgggttgctggctgaagcactacgttcctctgcagaccacaggtcctctggcctgaccggggtggatatgacatttatagccatggtcacgttccgcatacccactacggaggtgtggctgtcggtgaggtaacagaagcgactcccactgctctctgggccctgggacacccatggaaaggcctctgccaccagtttgagagcagccgtgctcccggcagtgaagatcacagtgtagtcttctgcggtggtgtggaagtgcgccaggattctgtagcgcacctgctccacagtgtcatgggtgagcttgctgctgatgttctggctgtgaggattaccataagtgttttccatgagatcactagtgaagctttcgagctggctctgggagaacaaggtggcacctgcatggtcaagatagacagttcctgccaggcggctgaactcgcgcgcccgcagctcgcgcaggctgcccgggccgtagccgtaggctagccgcggtgcgctcgggtcccgggaacccgcgaaggtccacagctcccgccctgactccgccgccgcgccggccatggccccggctagtccatccaggccggccgggcccgggaagtgc

SEQ ID NO: 11155 - RNA, 1612 nt, Homo sapiens
  source 1..1612: mol_type = other RNA
ctgaatagctgggactacaggtgcatgccaccatgcctggctaattttttatgttccatacagacagagtctcgtcaaatttcttggatggtttggaactcctgggctcaagcgatccttccgtctcagcctcccaaagtgcatattccattttgatgaaatactgtaatgctgataatttgtaaggatgcatttaccatccaatcagaaagattacaacatgatagatgactgctttggaaaatgctgctacttaatgatatgtgataaaaatgcttttagacatttggaatctaagacatgtactaaactacattcagcactcgatgtcaagcacaggaaaagaaaattcaaagatcttcagcataggagtgtgaaagatccatatccttaagatatcctcaaaagccaggaattactcatagtaagaaggtcataattaaaaatttcccttgtataccaggacaatgattaactgaagagctatactttatggaaaaatagacgaataccagcacatgctaaactaatggcctccatcttttcatattaccacttcatggtgcatatgtcctgccctttgcttcaaaatacactatggagccaaggaaactaagttcaaggaatagcagcaaatagggacttattcaacatacaatttaaaactattgttttaagtcagtggtttctaacatttcccccacattcacaccattctcaaattaaactacttaagtaaaagtagaaataaactctgaagaaaattagaatgtgcattctcacagagattatgatagtttcctaggtgtccccctccacccataaaactatacacaaatgcccacacccactaaactgggttgaatagtgtctcctcaaagctcatgtctacccagaacctcagaatgtaacattatttggaaatacttggcaaatgtgattagttaagatgaggacacactggatgaggatgagccctaaatcaaatcagtgatttccttacaagaagagacacacaaagaatgccatgtaaagatagaggcagagtttggagtgatgtgtgtatgtcttacaaggaaagtcaaggaactgcaggcaaccaccagaagctaggaagaggcaaagaaggattccctagaaccttcacaggaagtatgatcttgacaccttaattttgaacttctagcctccagaactgtgtaataagaaacacctgttattttaagccacaaaattagtggcttaaaatacagcggccctaggaaactaatatatccataaacatatgcacctaagaatcatagttattgcatgacttgtaatctctatttcaagtttctccttttccagttggaagtcctttgatgaattcaacctattgtaactaaggtaggcagcaaccttttccatactttccctactacacaaagtcctgccaatatctgaatttattacctcctttatccttgatagtactgggagatacgaatgcatcacatattcagataacccaatggcatttaggatggcagtaatcaaatttgggtggatcacgaggttaggagatcgagaccatcctggctaacacggtgaaaccccgtctctactaaac

SEQ ID NO: 11156 - RNA, 1453 nt, Homo sapiens
  source 1..1453: mol_type = other RNA
ctgaatagctgggactacaggtgcatgccaccatgcctggctaatttttttgtatttttagtagagacagggtttcacagtgttagccagtatggtctccatctcctgacctcatgatccgcctgcctcagcctcccaaagtgctgggattacaggcatgagccactgcacccagcctgcatttctgctttttaactttctagttacttgtatgtcctcgctttcgtacgtgcagtttggttgagagatgttagtggacagatgatggacatgaaagacgggttagaatgggagggaaatacacctgctatttttgtaccctagtatgtcctagtggtaaaaatgtgtcatatgcaactgcaaaagaaaggggaacatgttaaatgtcctagttttttctgttatctcaatgtgttgctctattcctattaagttttcctctcacatttactacaattagttctatattatcttgacaccattttctacgcttaaaacaacctcttccccctaactttaaaatcaggtacagtaaaagcctcttgttgaggatgtggttatcttggtagatgagagtgtgtcagaaacaggtagaaacttacctagcaaaagaactagtactgtatcttgacttgttatatggcaacaatcaattagatgataatttctatttaaaagcattctatatggggaaagacatgttcattttgataagtaaagacaaaatctaggtttttagttgatgtgtgttgtacatgtggtctttggaaagcaaaccaaactatgtattattgacattaaaaatgatgacttaatgctgggtaaatcctgtactcagaagatactcactgatgatccatccctgggtaaaccttctttgtctacactcattatctgtgatctcatccagtcttgtggctttaaatactatatggtgacaactacagccgagacctctcccctgaacttcagactcttctgtccagaagattatacaaattctctgtttggttatagaatttagaatgccccaaatcaagataattctccctcaattctgttcctcctataagcttccccaatcggtaaatgaaaactgtgtccttctagttaatcataccaaaatcctaaaaatcatccttaactcctctcatctctgatatccatatccaacccatgagcaaatactgtcaatctgccagaatccaaacatctctccagccccattgccaccaccctggtccaagccaccaccaggccttgcctagaatattgcaatacttttttttttttttttttttttttttttttttttgagacagagatggcatctcactctgttgcccaggatggagtacagtagctcaatcatagcttattacaacctccaactcctggatcaagcaatcctcccaactctgcgtcccgagtacctgggactataggcatgtgc

SEQ ID NO: 11157 - RNA, 4455 nt, Homo sapiens
  source 1..4455: mol_type = other RNA
ctgaatagctgggactacaggtgcatgccaccatgcctggttaatttttgtattttttgtagagacagggttgcccaggctggtcacgaactcctgagctcaagccatctgtctacctcggcctgcaaagtgctgggattacaggcataagccaacggccctggcttgattcatggcattttaatgaaaaatttcatgttttttcggtatgccaaagtgccatgtatgaaatatgaaatttggaagaatcgatgtaattgtacagccataggaaggcctcccttcaccatacaaaaaggtaacctttgctctattgctgccaccaagggccattttgtgggatgtggtaactttaagaatatttattacaattaaaaaaatcaaaatatgccatacttcataaacatcttatcagtaagttagaggtttaataaagaggttcaataaacagaaattttatttaacatatatttcaacatgaaatctataaattgcaaaggagcactgtgaattctttggaaaaacgtttgtttgctctactcacaagcttcatccttgtggcatgtattcagagctaggttatgtcctgctttttgtttaggcaggcataatgtctttcatggtattctcagaactctgttaaacttcactgctttgttaaatgtcactgctctgttaaacttcactgctcacaaaatctgagttaggacaaatgttcatgggggttgttgctcacatgttttcctatggctggttttcacaaaacggtatgcatctagtcctagggaagtacatgaaaggtcttcttagacggattctgctggaattatctcttgtctctgcagctgctggttctatcttctctcttctccagaagtggtattatttgtaaagtatttttgatggatgggtttttgcaaatggattcttgtatataatgtagtctttcactgagatcattaagggactctaggatcttctgttcttcagctgacagtgtgcagatgttgaattgttgagttttatttaaaggtagatttgatttctgtatctgtttgctattcaagacagtcagaatctcatcctccggcactgatgctttcactaagttttcagccatcaaaaactcagaagtactatctgaaacttcttcaatataagaagtaccccttgtagtttgttttggctcacttgaacttagcaggacactttgtccaaaattattaatttgctcactgtacttctgtcctacagatccagggttttgtcttttctgctctaaaatatttctccgcttagtttcagcaattcgttttcttctcataacagtagaccctgtagccctcttattttgatgcaggacattaggacctcttttccataagggaactgattcttcttcagcagttcttagagtcacagacggataactttcttcacaaacaggacttctttgggtgcaatataatgtcgcatcttgccgggcaactgcttgagtgccatttgaatgatttatttttgcgaaagtttggcactctgaagaacaatatgatggcagtgatggtatcacagtgactaggtcagaacaagcatttgagagtggagaactactttcctgattccactgattcaaactgtgttctgttggaagcacatgttttgaattaaaagagttatgtgtaataatgttttgaggattttcaggagttactggttgacactgagacacttgtatatttttaccacttctaatatttgatgtagattgaggaggaggacaaggtataattaattttccctgagcttgtgtaaatatgttgactttgcttgcagactgtggttgaatgacagcgccttttctgtttgtacatataaagcctgattggacttttgcagatcctggttttctaattatttttgctctacctctttgtggcttaccttgcttagttttagaatcatcatgtacagggattttactttcttctttttttgaggctggccaggcatgtttagcaaagttataacctgaaggtataaaacagttcaaaggcatatggtctgctccagatcctcctaaagtcgtaacattttcagagatagaatcctccctggacttctttgtatcagcagaatttacagcacaagtagaaacactaattatgttgcttccagcaccactttgaatgtggaattgttgagaatgctgttgagttgttcctgttttattcttcagtgaatgactgttttcagcattgttttctatattgctagtttcatcaaaccacctcagttttttaatggtctttggaatttctgcacctttttcctttgttaattcaatactatctctgatagctgctgctttttgatttccaaacttaaagctctgatttataattaatgccttaagataaccatgttcatatttagattctttctttaaaatacttttaagaaatctcacaccatttctctcatggatgttgtatttcattttcttatgctggccaacaaagtcataattagaagttacattagacaaggatgatgtttcagctaatttttgtttttcatcttttgaatcaggattgtgaggtatataggcatcttgaaaactgtctgaaaataaaggcaactcttccttattgcaattaaaatattttatctcttcttctttaccatctttcaattcatctaacttatcagaacactgcactgcatcaatttcttttatgtgtatactgttctttgctgaaggtctagctgactgtatattagatggcaaaactaaaggcgttgccactggtacacatgaagtaggaattgaagtagttccattttcttgatttaattcagaatatttctcttggtctggaaatgtagccacttcctgggttagagaatctgaagtgctttgggatttgctaaatttaaatgttgggctctcagtaactaatggtctctctcttttgaatgctccagaagtggagtcagttgtcctcatagtgctagtttcagaggtcttttcacattttttatctagtacaaacatgggtgggctagatacaaagggtactgaattattagcagtatttgtggctctttccactgttccattcaaaggagatggattttgttctttactattaaaatattcccatgaaggcagaacattagatttacttaaaatatctgagaaagctgtgacattctgagtatttgaagcatctaaatttgtaagccaattatttatatgttgagttttagagaatgccagtttatcttcatcaaagcagctgagattagttgattgcatatttgctggtttgagggaaatggtattccgctggatggatgtggaatgctccttattaagtgttaaatatatttcttcatgctctgtagcctcaagactgtctatacttgagagggtttcagaattggttatctgattaacttcatcacaaaatttttgcaaattgcttagatgttgatcttcgaggagtttctgagtttcctccagtttaagctggaacacatttttgctagtagccaaggttgccctcatgttttcattcatttctttctcacaattgattttggataagagttgtttctgatgcttgtgatcattttttgataatgcggaaggcaaggcagaatctatagctctccagtttattgttggtctacgggaaaagggaaggtttacttctgattttaagttggattcctgaatttgtttgagggcctcttctaatggaggaactggttttcgggaaactgctttcctccgctgtgaaagaggaacatgggcacgctggaatttttcagtaacttcttcaaacttctgttttctttgttgaagtatttgttctctaatttggtgttctttttcttcctgttcttttcgtttctcctcaaaagctttttttctccgatttgactccacaaaatatttacgtgctcgatttcgacatattttttgttgctgcagtaatatctggcgctcttcttctaaatttttctccagatggattttcatatctaggtaagagccaggtcggtgatgcccgccgctctcccgagggccgaggggggctctgtcgaggttgtccgatgattcagtgcccagttccccgaccgcgctccgggttccgggcctccccgccagcatccttcacttcagcgccgcctgtctgctcgcccccagaacctccctcatggcagctccggcttcctcctcctcctgctcggcccctccctacactccgtctctcaggccccgcgtcacgggcgcggaagggttggcctcgacagccctagctcccgcgcagcggcactggtgcctgtagcggcgatggcagctgaggcagcggcgacctcgccgggcaatagcagatggggcggcagcaaccctgcagccgccatcttgacaacaaccgacggcgc

SEQ ID NO: 11158 - RNA, 5137 nt, Homo sapiens
  source 1..5137: mol_type = other RNA
ctgaatagctgggactacaggtgcatgccaccatgcctggttaatttttgtattttttgtagagacagggttgcccaggctggtcacgaactcctgagctcaagccatctgtctacctcggcctgcaaagtgctgggattacaggcataagccaacggccctggcttgattcatggcattttaatgaaaaatttcatgttttttcggtatgccaaagtgccatgtatgaaatatgaaatttggaagaatcgatgtaattgtacagccataggaaggcctcccttcaccatacaaaaaggtaacctttgctctattgctgccaccaagggccattttgtgggatgtggtaactttaagaatatttattacaattaaaaaaatcaaaatatgccatacttcataaacatcttatcagtaagttagaggtttaataaagaggttcaataaacagaaattttatttaacatatatttcaacatgaaatctataaattgcaaaggagcactgtgaattctttggaaaaacgtttgtttgctctactcacaagcttcatccttgtggcatgtattcagagctaggttatgtcctgctttttgtttaggcaggcataatgtctttcatggtattctcagaactctgttaaacttcactgctttgttaaatgtcactgctctgttaaacttcactgctcacaaaatctgagttaggacaaatgttcatgggggttgttgctcacatgttttcctatggctggttttcacaaaacggtatgcatctagtcctagggaagtacatgaaaggtcttcttagacggattctgctggaattatctcttgtctctgcagctgctggttctatcttctctcttctccagaagtggtattatttgtaaagtatttttgatggatgggtttttgcaaatggattcttgtatataatgtagtctttcactgagatcattaagggactctaggatcttctgttcttcagctgacagtgtgcagatgttgaattgttgagttttatttaaaggtagatttgatttctgtatctgtttgctattcaagacagtcagaatctcatcctccggcactgatgctttcactaagttttcagccatcaaaaactcagaagtactatctgaaacttcttcaatataagaagtaccccttgtagtttgttttggctcacttgaacttagcaggacactttgtccaaaattattaatttgctcactgtacttctgtcctacagatccagggttttgtcttttctgctctaaaatatttctccgcttagtttcagcaattcgttttcttctcataacagtagaccctgtagccctcttattttgatgcaggacattaggacctcttttccataagggaactgattcttcttcagcagttcttagagtcacagacggataactttcttcacaaacaggacttctttgggtgcaatataatgtcgcatcttgccgggcaactgcttgagtgccatttgaatgatttatttttgcgaaagtttggcactctgaagaacaatatgatggcagtgatggtatcacagtgactaggtcagaacaagcatttgagagtggagaactactttcctgattccactgattcaaactgtgttctgttggaagcacatgttttgaattaaaagagttatgtgtaataatgttttgaggattttcaggagttactggttgacactgagacacttgtatatttttaccacttctaatatttgatgtagattgaggaggaggacaaggtataattaattttccctgagcttgtgtaaatatgttgactttgcttgcagactgtggttgaatgacagcgccttttctgtttgtacatataaagcctgattggacttttgcagatcctggttttctaattatttttgctctacctctttgtggcttaccttgcttagttttagaatcatcatgtacagggattttactttcttctttttttgaggctggccaggcatgtttagcaaagttataacctgaaggtataaaacagttcaaaggcatatggtctgctccagatcctcctaaagtcgtaacattttcagagatagaatcctccctggacttctttgtatcagcagaatttacagcacaagtagaaacactaattatgttgcttccagcaccactttgaatgtggaattgttgagaatgctgttgagttgttcctgttttattcttcagtgaatgactgttttcagcattgttttctatattgctagtttcatcaaaccacctcagttttttaatggtctttggaatttctgcacctttttcctttgttaattcaatactatctctgatagctgctgctttttgatttccaaacttaaagctctgatttataattaatgccttaagataaccatgttcatatttagattctttctttaaaatacttttaagaaatctcacaccatttctctcatggatgttgtatttcattttcttatgctggccaacaaagtcataattagaagttacattagacaaggatgatgtttcagctaatttttgtttttcatcttttgaatcaggattgtgaggtatataggcatcttgaaaactgtctgaaaataaaggcaactcttccttattgcaattaaaatattttatctcttcttctttaccatctttcaattcatctaacttatcagaacactgcactgcatcaatttcttttatgtgtatactgttctttgctgaaggtctagctgactgtatattagatggcaaaactaaaggcgttgccactggtacacatgaagtaggaattgaagtagttccattttcttgatttaattcagaatatttctcttggtctggaaatgtagccacttcctgggttagagaatctgaagtgctttgggatttgctaaatttaaatgttgggctctcagtaactaatggtctctctcttttgaatgctccagaagtggagtcagttgtcctcatagtgctagtttcagaggtcttttcacattttttatctagtacaaacatgggtgggctagatacaaagggtactgaattattagcagtatttgtggctctttccactgttccattcaaaggagatggattttgttctttactattaaaatattcccatgaaggcagaacattagatttacttaaaatatctgagaaagctgtgacattctgagtatttgaagcatctaaatttgtaagccaattatttatatgttgagttttagagaatgccagtttatcttcatcaaagcagctgagattagttgattgcatatttgctggtttgagggaaatggtattccgctggatggatgtggaatgctccttattaagtgttaaatatatttcttcatgctctgtagcctcaagactgtctatacttgagagggtttcagaattggttatctgattaacttcatcacaaaatttttgcaaattgcttagatgttgatcttcgaggagtttctgagtttcctccagtttaagctggaacacatttttgctagtagccaaggttgccctcatgttttcattcatttctttctcacaattgattttggataagagttgtttctgatgcttgtgatcattttttgataatgcggaaggcaaggcagaatctatagctctttaaagttgtcgtgtctcaactttcttctctattcctttcttctctactccactttcttctcttctcttctctactttcttcccccaatgaggaggattgaaggggtggataggaataaaaggagatggggaggtagaaacagaaggagagtgaagaatagggggaaaggaagaggaaatcataaaggaagaagaaacaggagaaactggagagggaaaagctaaataagttggaggcaaacctggagaggaagatgaatgcaaaggagaggaaaaaagagggatagatgaaggaggtaaggatggagaagtagaacaggaagtcgaagaagaggaaagaatagatgaggaggaagaaaacagtatacaggctgaagaaaaggatgtggaagtagaaggagatgaaggcaaagaagaagatggagaatgacagggagatgcaagggagagaactgaggctggtggatgatctgcaaaggcctcgggctgatttgacaatgctgtggcttgtggaacagattgctggactgactgaaaaggatccaagctagcaggatgtgcaggcaacggagtgacataagaaagagtggggactggtggataaggggggtgactggataaacaggaaggcttcaaaacagggagaggttccaaaggggttggggaaacaaccagtggagctccagtttattgttggtctacgggaaaagggaaggtttacttctgattttaagttggattcctgaatttgtttgagggcctcttctaatggaggaactggttttcgggaaactgctttcctccgctgtgaaagaggaacatgggcacgctggaatttttcagtaacttcttcaaacttctgttttctttgttgaagtatttgttctctaatttggtgttctttttcttcctgttcttttcgtttctcctcaaaagctttttttctccgatttgactccacaaaatatttacgtgctcgatttcgacatattttttgttgctgcagtaatatctggcgctcttcttctaaatttttctccagatggattttcatatctaggtaagagccaggtcggtgatgcccgccgctctcccgagggccgaggggggctctgtcgaggttgtccgatgattcagtgcccagttccccgaccgcgctccgggttccgggcctccccgccagcatccttcacttcagcgccgcctgtctgctcgcccccagaacctccctcatggcagctccggcttcctcctcctcctgctcggcccctccctacactccgtctctcaggccccgcgtcacgggcgcggaagggttggcctcgacagccctagctcccgcgcagcggcactggtgcctgtagcggcgatggcagctgaggcagcggcgacctcgccgggcaatagcagatggggcggcagcaaccctgcagccgccatcttgacaacaaccgacggcgc

SEQ ID NO: 11159 - RNA, 5536 nt, Homo sapiens
  source 1..5536: mol_type = other RNA
ctgaatagctgggactacaggtgcatgccacggtgcccagcctgttgctgttttatcagcactttaccaagttgtgtgcaatctttaatctctgagctaaacaactagcctgggtcaagcacatgttgcagcttccattgtcggagaagaaaatgagttagaaaacttattactgtatttactacattgaatatgcatgaccaatccttcattttcaagtaatcacagtgtcattataaactctaaattcactcagaagtgacttcttatcagaagtaaaaaaacaaagtttataattttagatgcctttgccttcttatgaagacatatgcagaattccatctctgactcgtttctggaccctggaaataactggctttttatagcaataactcaagggactgaatataatttaaaagtaatatacccaatacaggttgagcataccaaattccaaatttcaaaatccaaaatctgaaatactccaaaatctgaaagtttttgagcaccaacatgatgctcaaaggaaatgtttattgtagcatttaggattttagatttgggatgttcaactggtataatgcaaatattccaaaatccaaaatctaaaacacttacactcccaagcatttcagataagagatactcaaatcattaaagtacttattgagactattaggtgggtgctacaaaatcatttcccgacagaaatgtagggaatctcattctaatcaaattaaaactgtacatcaatgaaaaatacaacgttgaaaccgacaatccttcatccatggtaaatgaatgtcaatcaatttcccctcctgtgtctttgtttaaacgtctatgtaaagtctggagattttctgagcctatctctttggcaactcccactattttaattcacagtcctttcaagtccaagcaaatttctgagtttcacattgctctcctagttggataaatctttatatagaaagcacttacatttcagtaggagggtttagtcatttgtcaataaatgagatagctggttcaagcaatctaccaagtttatttctatgtgaaaatactgctagaagttagcaggtatacatgatctacatgattttaaattctttgtgaattctcaaaataaatctttagaaatatagtatactagaacatgtattataaaaattactttgcctgggtaatctaattcatcattgggcatacttagtatagccatatatacatacttataaacacaacttacaggtataagttgacataaatgaacataaactgacaatcaactaagaaggcaaagacatttaaataagcacattgtatttaaagagataaaaagctatcaactacctatcaaatgaatgttccaccagggggtgtagtatgcatttattatgtctgcagccaatttacctggcgtatgcacctaaaaacagttgaacaaaaagtatatttttgtagaatgatttatgacgtcccactggctttcatttttattccaaggaagctttgtctgtatattttattgcttttcaattaaatccaaagttatttccaacacttttggttttcaaattaaagctaagttgtaaagaaaactgtaaacaaatatctagattcttcagggaagtctgctattaatgctagattaattctttcctatagccaagaatcttttagcaaagcaattgtttcttagcgttaaatacaatctcacaaatattctacaaatggattttataggttgagatttcctttaagtaaagctcgtcgctaatgaatctggaaatattcagttattttaacaagaataatagcagctaacagtcattagtcccaaaataaagtgtttccttcaatctcagatttacaaaattggtttacctccacaaccacatttgatgaatgaaaacattttattagatatgttgattcactaagatgtgcgtattcacaaatttatccagcaatagatgtaacaagcatatgaaataataaatgagaacagtagcttttttccttgcaaaatgtacactctactgacatctatattgggtcagcatcacccagccactaagcaccaaagctgttgttgaacgcaggagtggctgatgctaaggctcaagctctggtgaaaacccacactgtgtggtcaggggagccggagcttctgccactgggaaactcttggtttctcctgactctccatctttaccttccccctcctggggaagaggacagccttgcctgttgttgctcttactgggggtaatgtgggaaggatgcctccaccaggaggtgccagtcatcatagagctccatggaaggcagcacagcacaggcggatgcaaaaagaatccaacatttcgagatgcattattcagtaactaggttacacatgaatacacactcaagatcaatttgtaaggaactatcaaaggcacagtcatgcatcgcttgacaacagggattcattctgagaaatgcgttgttgggtgaattcgtcgttgtgcaagcatcatagagtgcacttacacaaacctgggtggcacagcctgctacacacctagcctatatggtatggcctattgctcatagcctacaaaactgtgcagcatgttactgtactcaatactgtaggcaactgtaacacccctgcaacacacgggtaagtatgttgtgtatctgaacataccgaaacatagaaaaggtgcagtaaaaatacagcataaaaggttgaaaatggtccatctgtatagggctttttccatgaatggagtttgaaaaactggaaggtgctctgggtgagtcagtgagtgagtgctgagtgaaatgtgaaggcctaggacattaccgtacactactgtagactttataaacactatgcacttaagctacactaaattaataaaaatatttttctttcttcaataataagttaaccttagcttgctgcaccatttttactttatgaacttttaaagtttcttaactttttgactcttttgtaataacacttaaaacacaaacacattgtacaacacattgtacaaaaaagtctatatcctcttctgtgacctttttcctatttttaaggtttttaaatttttttcttacttttaaaacttttttgtcaaaattaagtcacaaacatacatattagcctaggcccacacagggccaggatcatcaatatcactgtcttctcctccacatctttttttttttttttttttttggatagagtctcactccgtcccccagactggagtccagtggcgcaatcttggctcactgcaacctctgcctcccaggttcaagcaattctcctgcctcagcctcctgagtagctgggattacaggtgcacgccaccatgcctgtctgatttttgtatttttagtacagacggcgtttcctcatgttggccaggctggtctccagctcctgatgtcaagtgatctgcccgtcttggcctcccaaagtgctgcaatcacaggcttgagccactacatctggcctcccctacatcttttcccactggaaggtcttcaagggcaattatatgcatgaagttgtcatctcctaggacaacaatgccatcttctggaacacctctggaaggatctgcctgaggctgttttacaggtaactttttaatatataagcagaaggaatatgctctaaaataacaataaaaattatagtatagtccaggggtatccaatgttttggcttccctgggtatactggaagaagaacaaaattgtcttgggtcacatataaaatacactaacactaacaatagctgatgagctaaaaaaaagaaaaaaagaaaaaaagaaaataaaaaggtccgtgcataaaactcatgttttaaaaaagtttacgaatttttgttgggccgcattcaaagccgtcctgggctgcatgcagcccgcagattggaccagcttggtatagtcaatacataaaccagtgacacaatcgctccttgtcattctcaactgttctgtattggacatacctgtatgtgctgggcttttatccgactggaagcacagtaggtttgccgacactaacatcaccacaggcagtgagtaatgccttgtgctatgacctcgtgatgaccaaaacattgttatgcggcacatgactatttctaagctcactagggcccctcgtgtcacacaacaggcatttgagagcctcagtctaacttctcacaagcaatctgcagcttctcaccaatgaagaaacaaaggcagccagggcacaacctttcatttccccaaggctgtgagaaagaggtggtataaacacaagtcttgtgtccccaaaagaagaatttattccttcttacattttggaaatattgatattttaaaaaaattactctgtgtgattttaggaatgtgagctgggctctgggaggcctgagtttaaactccgtctcttactcgctgtgttaacctctctgcatctcagtttccttctctgtaagacaagatgacgtcacaagacgcttcatatccctgcgcctcaaagaaaggcagtcatcacgcaatactgacttaatgggcccttcatcattttttggggataagaggtccaagacacatcttttgtgggaagatgagttttcccagtgatgctaagacactgggggatgggggtggaggtcaggttgggggtgggtttggggtagggaggtggaggcacacattaaaaaaaattgccaaaccaaatttattgctgatctcattttctcagcatttcttctacattcatcaaatattttagccactgccttttcatttcattttcctccagttgcacgtgctttgcttttgatgtggcacacactttgaaaatacattattaaacagatgagcctgtcacccctggagctggcactctgtcccctgcttattcttaacaaatctctctttgtgttcttttgtgctgaagtgattaatcatttccactatccaagggctgctgacaatctttctagatggctccgctgccatgacccctccccgcatccacacagtttgaaacatgctaggaatctgctgctgttcccggggctttattcccatcacagtgggctcctcatccatacggtaactagccaacctccaaaagagctccgcttttatttcttgcctttttccagagttcggggtgggggtgtgcgtgaaggggctcctggcgacttcagcaggaaaacaaggaaactcatttttctgggcagtatcctcctcttcactgcactgtggctgggttttcttctccccttcatgctttccctctggttatctgtaacaaagttttcaaatggctccatattgaaagcccaggctttgactcaccaggctctcaatctgtaatctggtttccagagctgcagcctaggtaggttttgggaagttgatctttttttaataagtgtttacaaacatttttaaactaactttaaaggtactattttaaaagcctatccttccccaaccccccgcccgc

SEQ ID NO: 11160 - RNA, 3451 nt, Homo sapiens
  source 1..3451: mol_type = other RNA
ctgaatagctgggactacaggtgcatgccactacacccagctaatttttgcatttttagtagacacagggtttcaccatgttggccaggctggtcttgaactcctgacctcaggtgatctgcccacctccgcctcccaaaatgctgggattacaagcatgagctactgcacctggtcagaaacagctattttaatagtgtcatctttaagaaagaaaaagttaagcggcaaaaatatgcttctgtatttagaaccatggacctttaattataactctaagactctatggattatttacaaaggaactaagaaaggcctaaacctgctgaagattatgaaggtagtcaatgacagaagacttgctagagctaagcattcttgtctctggtatagtgctatacgtcctcaactatgcctctgcagcaatagccttcctcttcatcttaggattaatggtactgagaaaatttaacatacagaatacaaaagtcactatcctattttcctaagaagaaaactttagaaatccatccaaccaaaacttaattttgccttttccttcagtgttcaagaagaaaaaaatgtatctagtagctctaagtggacagaaggacaagtgaaaactctagaatgcttaaacaagctataacaacaggtttgggcaccatctggtatcaccttactgaaactttccttagtaactcccctacaccccacaacaaaggacgagaaggaaggagctgaattcctactgttttggaggctgaaatgatgacccgtttgcctcccactccccctgctctgagggtatagagtagtgctttgccataaaaatgttagtgacacctaacagagctgagaccaacatctggggtattacagttgagaaaatcatggtgagaaaacaaagtcagatctacaggtcatccatagtctatactttataacagcctagactgtaaacaattttaatcacagaacattttcctgtctctaaagtgtatttataccgagttcagcattcaatctttccacagttccttcatgaatgttattttttttccctgctacatttataagctctttgaagttaataatcatgtctttaattttttgtattctcatgatatctatatattctaggcacagagtaaatactaaacatatacacattaatttactctcacagcagttaccataaaccaatgaaaccaaagtaatcatggggacgtgacaacagagattttctaataaagaaaaaaaataccaaaaaacccaccaatgctgtaatttcaagaatcctgtcgtgataaaagaagcaagtggagttgggctttcctagaaccttctttgccctaccttcacagattatccttagtataaacttgcagtgtgttaaaactcaggtatctatgttttatacagaaacttgcaaggtaacgaccaaaatatctcagtgcaattaaatttacaaattcttcccattaaaagaactacatgggaattccctgtgataatttctcaaagttctcattaaaaacttaagaaaaaggtaaataaaccaaacatcttcatagaaaaattgtatttacaactccattcaaaagcagtttttaaaagcaaacacaatgtaacactgaaggtgaaaaatctaagctcacccaaagctgccaggtctaataaattactgacagaatactgtatcaaaaataaggcaataaccgaaaatataccattaaagatttctccatccccacaactagatagaatgaatctatctaggagcaaatgacatgctttattcagtttcaccatgtctgaaacctttaaggacagaagtgataaaatgttatcttcattcttcattagacttgaacacttgaaggaaaataatttctaaagcacaaagaggtaaagaagtataatctttcaaaaagatattcagtgttcaaaattcaagaatgcaatatcaatacacaatgggcattaggtgaatatacacaatacgatgagagcaaattaatttatttagtactttttccattccatatcatcaggaggattgatttcaactttccttttacctacatcagaccagttggtactcaaaactgtaccacccgactccataaaggatttgttcatggcacgtttcacttcatcagaaccatctgaatagatctgctgaaataatctgtttaaagctgcatctccctccaacttttcattcttttcttcttctttgatctcaccaaccaatttatcccaatttcttgtataaggagatgatgatggatataggttctttacatctgctacgaattgttttggcgtaggcacatctccttgcccctctagcttttcccatctcacagcctctggctttttcagtttaatttcaatctttgttgaaagtactttaaacgtgctctgttctggtattataggatgaagaagttccagtttcaaattgtaatcctctccagaaggaagtttaaccaaagcagacaactctttttctgaaaattccacatttacatcattcttctgaacattcttgatcataagtgtaatgactacttgagattctgtttgataccagtcatacttgatttttgactgatgagtccacacctcagattctgagccattctgagcttcttgacaccttttaatccagacactgaaattagcatctgcacctgtaatcccagcactttgggagtccaaggcaggtggatcacttgaggtcaagagttggagaccagcctggccaacacgatgaaaccccgtctctatatctaatttttgtccttctgtaaaagtttctagggcagcagcatagtttttttcatggtattcacatattccttttctcagcatagcagtggaattatttggattgagttctagagacttctttgcatcagcaacagcaacacagtaattcccaagaagaatgtgacaataagctctttgacaataatactgtgcatcatctggtttctgttccaaagccttagtcagctccggagctgagacgcagcatcaacaagagcctgggtccctgtccggcggtgcggggagaaggcgggtcagcggggacccgaagtggcccagctcccctaagaagagtggaggaagcagaaatgggctctctcacctctaacgccgcctgggggtcctcgtcgattagggcatccgagaagctctggaaaaacctctgggatgttgcagttcctgctgcagccgccgccatccctcgtagtcgctgttgctgccgccggagctgctactatcacggttaccacctccaccaccgcccaagggggaaacttctggagaaacaccaaccgagcttccgtcctaaatagccagcgagcagccacgcagcgtgctgctagggggacgggaggcgacacgccggcgcggggccggctgggacagtgga

SEQ ID NO: 11161 - RNA, 3211 nt, Homo sapiens
  source 1..3211: mol_type = other RNA
ctgaatagctgggactacaggtgcatgccactacacccagctaatttttgcatttttagtagacacagggtttcaccatgttggccaggctggtcttgaactcctgacctcaggtgatctgcccacctccgcctcccaaaatgctgggattacaagcatgagctactgcacctggtcagaaacagctattttaatagtgtcatctttaagaaagaaaaagttaagcggcaaaaatatgcttctgtatttagaaccatggacctttaattataactctaagactctatggattatttacaaaggaactaagaaaggcctaaacctgctgaagattatgaaggtagtcaatgacagaagacttgctagagctaagcattcttgtctctggtatagtgctatacgtcctcaactatgcctctgcagcaatagccttcctcttcatcttaggattaatggtactgagaaaatttaacatacagaatacaaaagtcactatcctattttcctaagaagaaaactttagaaatccatccaaccaaaacttaattttgccttttccttcagtgttcaagaagaaaaaaatgtatctagtagctctaagtggacagaaggacaagtgaaaactctagaatgcttaaacaagctataacaacaggtttgggcaccatctggtatcaccttactgaaactttccttagtaactcccctacaccccacaacaaaggacgagaaggaaggagctgaattcctactgttttggaggctgaaatgatgacccgtttgcctcccactccccctgctctgagggtatagagtagtgctttgccataaaaatgttagtgacacctaacagagctgagaccaacatctggggtattacagttgagaaaatcatggtgagaaaacaaagtcagatctacaggtcatccatagtctatactttataacagcctagactgtaaacaattttaatcacagaacattttcctgtctctaaagtgtatttataccgagttcagcattcaatctttccacagttccttcatgaatgttattttttttccctgctacatttataagctctttgaagttaataatcatgtctttaattttttgtattctcatgatatctatatattctaggcacagagtaaatactaaacatatacacattaatttactctcacagcagttaccataaaccaatgaaaccaaagtaatcatggggacgtgacaacagagattttctaataaagaaaaaaaataccaaaaaacccaccaatgctgtaatttcaagaatcctgtcgtgataaaagaagcaagtggagttgggctttcctagaaccttctttgccctaccttcacagattatccttagtataaacttgcagtgtgttaaaactcaggtatctatgttttatacagaaacttgcaaggtaacgaccaaaatatctcagtgcaattaaatttacaaattcttcccattaaaagaactacatgggaattccctgtgataatttctcaaagttctcattaaaaacttaagaaaaaggtaaataaaccaaacatcttcatagaaaaattgtatttacaactccattcaaaagcagtttttaaaagcaaacacaatgtaacactgaaggtgaaaaatctaagctcacccaaagctgccaggtctaataaattactgacagaatactgtatcaaaaataaggcaataaccgaaaatataccattaaagatttctccatccccacaactagatagaatgaatctatctaggagcaaatgacatgctttattcagtttcaccatgtctgaaacctttaaggacagaagtgataaaatgttatcttcattcttcattagacttgaacacttgaaggaaaataatttctaaagcacaaagaggtaaagaagtataatctttcaaaaagatattcagtgttcaaaattcaagaatgcaatatcaatacacaatgggcattaggtgaatatacacaatacgatgagagcaaattaatttatttagtactttttccattccatatcatcaggaggattgatttcaactttccttttacctacatcagaccagttggtactcaaaactgtaccacccgactccataaaggatttgttcatggcacgtttcacttcatcagaaccatctgaatagatctgctgaaataatctgtttaaagctgcatctccctccaacttttcattcttttcttcttctttgatctcaccaaccaatttatcccaatttcttgtataaggagatgatgatggatataggttctttacatctgctacgaattgttttggcgtaggcacatctccttgcccctctagcttttcccatctcacagcctctggctttttcagtttaatttcaatctttgttgaaagtactttaaacgtgctctgttctggtattataggatgaagaagttccagtttcaaattgtaatcctctccagaaggaagtttaaccaaagcagacaactctttttctgaaaattccacatttacatcattcttctgaacattcttgatcataagtgtaatgactacttgagattctgtttgataccagtcatacttgatttttgactgatgagtccacacctcagattctgagccattctgagcttcttgacaccttttaatccagacactgaaattagcatctgcacctgtaatcccagcactttgggagtccaaggcaggtggatcacttgaggtcaagagttggagaccagcctggccaacacgatgaaaccccgtctctatatctaatttttgtccttctgtaaaagtttctagggcagcagcatagtttttttcatggtattcacatattccttttctcagcatagcagtggaattatttggattgagttctagagacttctttgcatcagcaacagcaacacagtaattcccaagaagaatgtgacaataagctctttgacaataatactgtgcatcatctggtttctgttccaaagccttagtcagctcctctaacgccgcctgggggtcctcgtcgattagggcatccgagaagctctggaaaaacctctgggatgttgcagttcctgctgcagccgccgccatccctcgtagtcgctgttgctgccgccggagctgctactatcacggttaccacctccaccaccgcccaagggggaaacttctggag

SEQ ID NO: 11162 - RNA, 3250 nt, Homo sapiens
  source 1..3250: mol_type = other RNA
ctgaatagctgggactacaggtgcatgccactacacccagctaatttttgcatttttagtagacacagggtttcaccatgttggccaggctggtcttgaactcctgacctcaggtgatctgcccacctccgcctcccaaaatgctgggattacaagcatgagctactgcacctggtcagaaacagctattttaatagtgtcatctttaagaaagaaaaagttaagcggcaaaaatatgcttctgtatttagaaccatggacctttaattataactctaagactctatggattatttacaaaggaactaagaaaggcctaaacctgctgaagattatgaaggtagtcaatgacagaagacttgctagagctaagcattcttgtctctggtatagtgctatacgtcctcaactatgcctctgcagcaatagccttcctcttcatcttaggattaatggtactgagaaaatttaacatacagaatacaaaagtcactatcctattttcctaagaagaaaactttagaaatccatccaaccaaaacttaattttgccttttccttcagtgttcaagaagaaaaaaatgtatctagtagctctaagtggacagaaggacaagtgaaaactctagaatgcttaaacaagctataacaacaggtttgggcaccatctggtatcaccttactgaaactttccttagtaactcccctacaccccacaacaaaggacgagaaggaaggagctgaattcctactgttttggaggctgaaatgatgacccgtttgcctcccactccccctgctctgagggtatagagtagtgctttgccataaaaatgttagtgacacctaacagagctgagaccaacatctggggtattacagttgagaaaatcatggtgagaaaacaaagtcagatctacaggtcatccatagtctatactttataacagcctagactgtaaacaattttaatcacagaacattttcctgtctctaaagtgtatttataccgagttcagcattcaatctttccacagttccttcatgaatgttattttttttccctgctacatttataagctctttgaagttaataatcatgtctttaattttttgtattctcatgatatctatatattctaggcacagagtaaatactaaacatatacacattaatttactctcacagcagttaccataaaccaatgaaaccaaagtaatcatggggacgtgacaacagagattttctaataaagaaaaaaaataccaaaaaacccaccaatgctgtaatttcaagaatcctgtcgtgataaaagaagcaagtggagttgggctttcctagaaccttctttgccctaccttcacagattatccttagtataaacttgcagtgtgttaaaactcaggtatctatgttttatacagaaacttgcaaggtaacgaccaaaatatctcagtgcaattaaatttacaaattcttcccattaaaagaactacatgggaattccctgtgataatttctcaaagttctcattaaaaacttaagaaaaaggtaaataaaccaaacatcttcatagaaaaattgtatttacaactccattcaaaagcagtttttaaaagcaaacacaatgtaacactgaaggtgaaaaatctaagctcacccaaagctgccaggtctaataaattactgacagaatactgtatcaaaaataaggcaataaccgaaaatataccattaaagatttctccatccccacaactagatagaatgaatctatctaggagcaaatgacatgctttattcagtttcaccatgtctgaaacctttaaggacagaagtgataaaatgttatcttcattcttcattagacttgaacacttgaaggaaaataatttctaaagcacaaagaggtaaagaagtataatctttcaaaaagatattcagtgttcaaaattcaagaatgcaatatcaatacacaatgggcattaggtgaatatacacaatacgatgagagcaaattaatttatttagtactttttccattccatatcatcaggaggattgatttcaactttccttttacctacatcagaccagttggtactcaaaactgtaccacccgactccataaaggatttgttcatggcacgtttcacttcatcagaaccatctgaatagatctgctgaaataatctgtttaaagctgcatctccctccaacttttcattcttttcttcttctttgatctcaccaaccaatttatcccaatttcttgtataaggagatgatgatggatataggttctttacatctgctacgaattgttttggcgtaggcacatctccttgcccctctagcttttcccatctcacagcctctggctttttcagtttaatttcaatctttgttgaaagtactttaaacgtgctctgttctggtattataggatgaagaagttccagtttcaaattgtaatcctctccagaaggaagtttaaccaaagcagacaactctttttctgaaaattccacatttacatcattcttctgaacattcttgatcataagtgtaatgactacttgagattctgtttgataccagtcatacttgatttttgactgatgagtccacacctcagattctgagccattctgagcttcttgacaccttttaatccagacactgaaattagcatctgcacctgtaatcccagcactttgggagtccaaggcaggtggatcacttgaggtcaagagttggagaccagcctggccaacacgatgaaaccccgtctctatatctaatttttgtccttctgtaaaagtttctagggcagcagcatagtttttttcatggtattcacatattccttttctcagcatagcagtggaattatttggattgagttctagagacttctttgcatcagcaacagcaacttccttttggcttaacatttagcttccttcttaaagctcttcaatgaatacagctgtgtcacaaaattcacctccttgtctcattaacattttctatgtaattttactcaaggtattcagtttttcccacagtaattcccaagaagaatgtgacaataagctctttgacaataatactgtgcatcatctggtttctgttccaaagccttagtcagctccggagctgagacgcagcatcaacaagagcctgggtccctgtccggcggtgcggggagaaggcgggtcagcggggacccgaagtggcccagct

SEQ ID NO: 11163 - RNA, 3331 nt, Homo sapiens
  source 1..3331: mol_type = other RNA
ctgaatagctgggactacaggtgcatgccactacacccagctaatttttgcatttttagtagacacagggtttcaccatgttggccaggctggtcttgaactcctgacctcaggtgatctgcccacctccgcctcccaaaatgctgggattacaagcatgagctactgcacctggtcagaaacagctattttaatagtgtcatctttaagaaagaaaaagttaagcggcaaaaatatgcttctgtatttagaaccatggacctttaattataactctaagactctatggattatttacaaaggaactaagaaaggcctaaacctgctgaagattatgaaggtagtcaatgacagaagacttgctagagctaagcattcttgtctctggtatagtgctatacgtcctcaactatgcctctgcagcaatagccttcctcttcatcttaggattaatggtactgagaaaatttaacatacagaatacaaaagtcactatcctattttcctaagaagaaaactttagaaatccatccaaccaaaacttaattttgccttttccttcagtgttcaagaagaaaaaaatgtatctagtagctctaagtggacagaaggacaagtgaaaactctagaatgcttaaacaagctataacaacaggtttgggcaccatctggtatcaccttactgaaactttccttagtaactcccctacaccccacaacaaaggacgagaaggaaggagctgaattcctactgttttggaggctgaaatgatgacccgtttgcctcccactccccctgctctgagggtatagagtagtgctttgccataaaaatgttagtgacacctaacagagctgagaccaacatctggggtattacagttgagaaaatcatggtgagaaaacaaagtcagatctacaggtcatccatagtctatactttataacagcctagactgtaaacaattttaatcacagaacattttcctgtctctaaagtgtatttataccgagttcagcattcaatctttccacagttccttcatgaatgttattttttttccctgctacatttataagctctttgaagttaataatcatgtctttaattttttgtattctcatgatatctatatattctaggcacagagtaaatactaaacatatacacattaatttactctcacagcagttaccataaaccaatgaaaccaaagtaatcatggggacgtgacaacagagattttctaataaagaaaaaaaataccaaaaaacccaccaatgctgtaatttcaagaatcctgtcgtgataaaagaagcaagtggagttgggctttcctagaaccttctttgccctaccttcacagattatccttagtataaacttgcagtgtgttaaaactcaggtatctatgttttatacagaaacttgcaaggtaacgaccaaaatatctcagtgcaattaaatttacaaattcttcccattaaaagaactacatgggaattccctgtgataatttctcaaagttctcattaaaaacttaagaaaaaggtaaataaaccaaacatcttcatagaaaaattgtatttacaactccattcaaaagcagtttttaaaagcaaacacaatgtaacactgaaggtgaaaaatctaagctcacccaaagctgccaggtctaataaattactgacagaatactgtatcaaaaataaggcaataaccgaaaatataccattaaagatttctccatccccacaactagatagaatgaatctatctaggagcaaatgacatgctttattcagtttcaccatgtctgaaacctttaaggacagaagtgataaaatgttatcttcattcttcattagacttgaacacttgaaggaaaataatttctaaagcacaaagaggtaaagaagtataatctttcaaaaagatattcagtgttcaaaattcaagaatgcaatatcaatacacaatgggcattaggtgaatatacacaatacgatgagagcaaattaatttatttagtactttttccattccatatcatcaggaggattgatttcaactttccttttacctacatcagaccagttggtactcaaaactgtaccacccgactccataaaggatttgttcatggcacgtttcacttcatcagaaccatctgaatagatctgctgaaataatctgtttaaagctgcatctccctccaacttttcattcttttcttcttctttgatctcaccaaccaatttatcccaatttcttgtataaggagatgatgatggatataggttctttacatctgctacgaattgttttggcgtaggcacatctccttgcccctctagcttttcccatctcacagcctctggctttttcagtttaatttcaatctttgttgaaagtactttaaacgtgctctgttctggtattataggatgaagaagttccagtttcaaattgtaatcctctccagaaggaagtttaaccaaagcagacaactctttttctgaaaattccacatttacatcattcttctgaacattcttgatcataagtgtaatgactacttgagattctgtttgataccagtcatacttgatttttgactgatgagtccacacctcagattctgagccattctgagcttcttgacaccttttaatccagacactgaaattagcatctgcacctgtaatcccagcactttgggagtccaaggcaggtggatcacttgaggtcaagagttggagaccagcctggccaacacgatgaaaccccgtctctatatctaatttttgtccttctgtaaaagtttctagggcagcagcatagtttttttcatggtattcacatattccttttctcagcatagcagtggaattatttggattgagttctagagacttctttgcatcagcaacagcaacttccttttggcttaacatttagcttccttcttaaagctcttcaatgaatacagctgtgtcacaaaattcacctccttgtctcattaacattttctatgtaattttactcaaggtattcagtttttcccacagtaattcccaagaagaatgtgacaataagctctttgacaataatactgtgcatcatctggtttctgttccaaagccttagtcagctcctctaacgccgcctgggggtcctcgtcgattagggcatccgagaagctctggaaaaacctctgggatgttgcagttcctgctgcagccgccgccatccctcgtagtcgctgttgctgccgccggagctgctactatcacggttaccacctccaccaccgcccaagggggaaac

SEQ ID NO: 11164 - RNA, 3262 nt, Homo sapiens
  source 1..3262: mol_type = other RNA
ctgaatagctgggactacaggtgcatgccactacacccagctaatttttgcatttttagtagacacagggtttcaccatgttggccaggctggtcttgaactcctgacctcaggtgatctgcccacctccgcctcccaaaatgctgggattacaagcatgagctactgcacctggtcagaaacagctattttaatagtgtcatctttaagaaagaaaaagttaagcggcaaaaatatgcttctgtatttagaaccatggacctttaattataactctaagactctatggattatttacaaaggaactaagaaaggcctaaacctgctgaagattatgaaggtagtcaatgacagaagacttgctagagctaagcattcttgtctctggtatagtgctatacgtcctcaactatgcctctgcagcaatagccttcctcttcatcttaggattaatggtactgagaaaatttaacatacagaatacaaaagtcactatcctattttcctaagaagaaaactttagaaatccatccaaccaaaacttaattttgccttttccttcagtgttcaagaagaaaaaaatgtatctagtagctctaagtggacagaaggacaagtgaaaactctagaatgcttaaacaagctataacaacaggtttgggcaccatctggtatcaccttactgaaactttccttagtaactcccctacaccccacaacaaaggacgagaaggaaggagctgaattcctactgttttggaggctgaaatgatgacccgtttgcctcccactccccctgctctgagggtatagagtagtgctttgccataaaaatgttagtgacacctaacagagctgagaccaacatctggggtattacagttgagaaaatcatggtgagaaaacaaagtcagatctacaggtcatccatagtctatactttataacagcctagactgtaaacaattttaatcacagaacattttcctgtctctaaagtgtatttataccgagttcagcattcaatctttccacagttccttcatgaatgttattttttttccctgctacatttataagctctttgaagttaataatcatgtctttaattttttgtattctcatgatatctatatattctaggcacagagtaaatactaaacatatacacattaatttactctcacagcagttaccataaaccaatgaaaccaaagtaatcatggggacgtgacaacagagattttctaataaagaaaaaaaataccaaaaaacccaccaatgctgtaatttcaagaatcctgtcgtgataaaagaagcaagtggagttgggctttcctagaaccttctttgccctaccttcacagattatccttagtataaacttgcagtgtgttaaaactcaggtatctatgttttatacagaaacttgcaaggtaacgaccaaaatatctcagtgcaattaaatttacaaattcttcccattaaaagaactacatgggaattccctgtgataatttctcaaagttctcattaaaaacttaagaaaaaggtaaataaaccaaacatcttcatagaaaaattgtatttacaactccattcaaaagcagtttttaaaagcaaacacaatgtaacactgaaggtgaaaaatctaagctcacccaaagctgccaggtctaataaattactgacagaatactgtatcaaaaataaggcaataaccgaaaatataccattaaagatttctccatccccacaactagatagaatgaatctatctaggagcaaatgacatgctttattcagtttcaccatgtctgaaacctttaaggacagaagtgataaaatgttatcttcattcttcattagacttgaacacttgaaggaaaataatttctaaagcacaaagaggtaaagaagtataatctttcaaaaagatattcagtgttcaaaattcaagaatgcaatatcaatacacaatgggcattaggtgaatatacacaatacgatgagagcaaattaatttatttagtactttttccattccatatcatcaggaggattgatttcaactttccttttacctacatcagaccagttggtactcaaaactgtaccacccgactccataaaggatttgttcatggcacgtttcacttcatcagaaccatctgaatagatctgctgaaataatctgtttaaagctgcatctccctccaacttttcattcttttcttcttctttgatctcaccaaccaatttatcccaatttcttgtataaggagatgatgatggatataggttctttacatctgctacgaattgttttggcgtaggcacatctccttgcccctctagcttttcccatctcacagcctctggctttttcagtttaatttcaatctttgttgaaagtactttaaacgtgctctgttctggtattataggatgaagaagttccagtttcaaattgtaatcctctccagaaggaagtttaaccaaagcagacaactctttttctgaaaattccacatttacatcattcttctgaacattcttgatcataagtgtaatgactacttgagattctgtttgataccagtcatacttgatttttgactgatgagtccacacctcagattctgagccattctgagcttcttgacaccttttaatccagacactgaaattagcatctgcacctgtaatcccagcactttgggagtccaaggcaggtggatcacttgaggtcaagagttggagaccagcctggccaacacgatgaaaccccgtcttatctaatttttgtccttctgtaaaagtttctagggcagcagcatagtttttttcatggtattcacatattccttttctcagcatagcagtggaattatttggattgagttctagagacttctttgcatcagcaacagcaacacagtaattcccaagaagaatgtgacaataagctctttgacaataatactgtgcatcatctggtttctgttccaaagccttagtcagctccggagctgagacgcagcatcaacaagagcctgggtccctgtccggcggtgcggggagaaggcgggtcagcggggacccgaagtggcccagctcccctaagaagagtggaggaagcagaaatgggctctctcacctctaacgccgcctgggggtcctcgtcgattagggcatccgagaagctctggaaaaacctctgggatgttgcagttcctgctgcagccgccgccatccctcg

SEQ ID NO: 11165 - RNA, 3341 nt, Homo sapiens
  source 1..3341: mol_type = other RNA
ctgaatagctgggactacaggtgcatgccactacacccagctaatttttgcatttttagtagacacagggtttcaccatgttggccaggctggtcttgaactcctgacctcaggtgatctgcccacctccgcctcccaaaatgctgggattacaagcatgagctactgcacctggtcagaaacagctattttaatagtgtcatctttaagaaagaaaaagttaagcggcaaaaatatgcttctgtatttagaaccatggacctttaattataactctaagactctatggattatttacaaaggaactaagaaaggcctaaacctgctgaagattatgaaggtagtcaatgacagaagacttgctagagctaagcattcttgtctctggtatagtgctatacgtcctcaactatgcctctgcagcaatagccttcctcttcatcttaggattaatggtactgagaaaatttaacatacagaatacaaaagtcactatcctattttcctaagaagaaaactttagaaatccatccaaccaaaacttaattttgccttttccttcagtgttcaagaagaaaaaaatgtatctagtagctctaagtggacagaaggacaagtgaaaactctagaatgcttaaacaagctataacaacaggtttgggcaccatctggtatcaccttactgaaactttccttagtaactcccctacaccccacaacaaaggacgagaaggaaggagctgaattcctactgttttggaggctgaaatgatgacccgtttgcctcccactccccctgctctgagggtatagagtagtgctttgccataaaaatgttagtgacacctaacagagctgagaccaacatctggggtattacagttgagaaaatcatggtgagaaaacaaagtcagatctacaggtcatccatagtctatactttataacagcctagactgtaaacaattttaatcacagaacattttcctgtctctaaagtgtatttataccgagttcagcattcaatctttccacagttccttcatgaatgttattttttttccctgctacatttataagctctttgaagttaataatcatgtctttaattttttgtattctcatgatatctatatattctaggcacagagtaaatactaaacatatacacattaatttactctcacagcagttaccataaaccaatgaaaccaaagtaatcatggggacgtgacaacagagattttctaataaagaaaaaaaataccaaaaaacccaccaatgctgtaatttcaagaatcctgtcgtgataaaagaagcaagtggagttgggctttcctagaaccttctttgccctaccttcacagattatccttagtataaacttgcagtgtgttaaaactcaggtatctatgttttatacagaaacttgcaaggtaacgaccaaaatatctcagtgcaattaaatttacaaattcttcccattaaaagaactacatgggaattccctgtgataatttctcaaagttctcattaaaaacttaagaaaaaggtaaataaaccaaacatcttcatagaaaaattgtatttacaactccattcaaaagcagtttttaaaagcaaacacaatgtaacactgaaggtgaaaaatctaagctcacccaaagctgccaggtctaataaattactgacagaatactgtatcaaaaataaggcaataaccgaaaatataccattaaagatttctccatccccacaactagatagaatgaatctatctaggagcaaatgacatgctttattcagtttcaccatgtctgaaacctttaaggacagaagtgataaaatgttatcttcattcttcattagacttgaacacttgaaggaaaataatttctaaagcacaaagaggtaaagaagtataatctttcaaaaagatattcagtgttcaaaattcaagaatgcaatatcaatacacaatgggcattaggtgaatatacacaatacgatgagagcaaattaatttatttagtactttttccattccatatcatcaggaggattgatttcaactttccttttacctacatcagaccagttggtactcaaaactgtaccacccgactccataaaggatttgttcatggcacgtttcacttcatcagaaccatctgaatagatctgctgaaataatctgtttaaagctgcatctccctccaacttttcattcttttcttcttctttgatctcaccaaccaatttatcccaatttcttgtataaggagatgatgatggatataggttctttacatctgctacgaattgttttggcgtaggcacatctccttgcccctctagcttttcccatctcacagcctctggctttttcagtttaatttcaatctttgttgaaagtactttaaacgtgctctgttctggtattataggatgaagaagttccagtttcaaattgtaatcctctccagaaggaagtttaaccaaagcagacaactctttttctgaaaattccacatttacatcattcttctgaacattcttgatcataagtgtaatgactacttgagattctgtttgataccagtcatacttgatttttgactgatgagtccacacctcagattctgagccattctgagcttcttgacaccttttaatccagacactgaaattagcatctgcacctgtaatcccagcactttgggagtccaaggcaggtggatcacttgaggtcaagagttggagaccagcctggccaacacgatgaaaccccgtcttatctaatttttgtccttctgtaaaagtttctagggcagcagcatagtttttttcatggtattcacatattccttttctcagcatagcagtggaattatttggattgagttctagagacttctttgcatcagcaacagcaacacagtaattcccaagaagaatgtgacaataagctctttgacaataatactgtgcatcatctggtttctgttccaaagccttagtcagctcctctaacgccgcctgggggtcctcgtcgattagggcatccgagaagctctggaaaaacctctgggatgttgcagttcctgctgcagccgccgccatccctcgtagtcgctgttgctgccgccggagctgctactatcacggttaccacctccaccaccgcccaagggggaaacttctggagaaacaccaaccgagcttccgtcctaaatagccagcgagcagccacgcagcgtgctgctagggggacgggaggcgacacgccggcgcggggccggctgggacagtggaggaccgattcctcccagccgcacccc

SEQ ID NO: 11166 - RNA, 3351 nt, Homo sapiens
  source 1..3351: mol_type = other RNA
ctgaatagctgggactacaggtgcatgccactacacccagctaatttttgcatttttagtagacacagggtttcaccatgttggccaggctggtcttgaactcctgacctcaggtgatctgcccacctccgcctcccaaaatgctgggattacaagcatgagctactgcacctggtcagaaacagctattttaatagtgtcatctttaagaaagaaaaagttaagcggcaaaaatatgcttctgtatttagaaccatggacctttaattataactctaagactctatggattatttacaaaggaactaagaaaggcctaaacctgctgaagattatgaaggtagtcaatgacagaagacttgctagagctaagcattcttgtctctggtatagtgctatacgtcctcaactatgcctctgcagcaatagccttcctcttcatcttaggattaatggtactgagaaaatttaacatacagaatacaaaagtcactatcctattttcctaagaagaaaactttagaaatccatccaaccaaaacttaattttgccttttccttcagtgttcaagaagaaaaaaatgtatctagtagctctaagtggacagaaggacaagtgaaaactctagaatgcttaaacaagctataacaacaggtttgggcaccatctggtatcaccttactgaaactttccttagtaactcccctacaccccacaacaaaggacgagaaggaaggagctgaattcctactgttttggaggctgaaatgatgacccgtttgcctcccactccccctgctctgagggtatagagtagtgctttgccataaaaatgttagtgacacctaacagagctgagaccaacatctggggtattacagttgagaaaatcatggtgagaaaacaaagtcagatctacaggtcatccatagtctatactttataacagcctagactgtaaacaattttaatcacagaacattttcctgtctctaaagtgtatttataccgagttcagcattcaatctttccacagttccttcatgaatgttattttttttccctgctacatttataagctctttgaagttaataatcatgtctttaattttttgtattctcatgatatctatatattctaggcacagagtaaatactaaacatatacacattaatttactctcacagcagttaccataaaccaatgaaaccaaagtaatcatggggacgtgacaacagagattttctaataaagaaaaaaaataccaaaaaacccaccaatgctgtaatttcaagaatcctgtcgtgataaaagaagcaagtggagttgggctttcctagaaccttctttgccctaccttcacagattatccttagtataaacttgcagtgtgttaaaactcaggtatctatgttttatacagaaacttgcaaggtaacgaccaaaatatctcagtgcaattaaatttacaaattcttcccattaaaagaactacatgggaattccctgtgataatttctcaaagttctcattaaaaacttaagaaaaaggtaaataaaccaaacatcttcatagaaaaattgtatttacaactccattcaaaagcagtttttaaaagcaaacacaatgtaacactgaaggtgaaaaatctaagctcacccaaagctgccaggtctaataaattactgacagaatactgtatcaaaaataaggcaataaccgaaaatataccattaaagatttctccatccccacaactagatagaatgaatctatctaggagcaaatgacatgctttattcagtttcaccatgtctgaaacctttaaggacagaagtgataaaatgttatcttcattcttcattagacttgaacacttgaaggaaaataatttctaaagcacaaagaggtaaagaagtataatctttcaaaaagatattcagtgttcaaaattcaagaatgcaatatcaatacacaatgggcattaggtgaatatacacaatacgatgagagcaaattaatttatttagtactttttccattccatatcatcaggaggattgatttcaactttccttttacctacatcagaccagttggtactcaaaactgtaccacccgactccataaaggatttgttcatggcacgtttcacttcatcagaaccatctgaatagatctgctgaaataatctgtttaaagctgcatctccctccaacttttcattcttttcttcttctttgatctcaccaaccaatttatcccaatttcttgtataaggagatgatgatggatataggttctttacatctgctacgaattgttttggcgtaggcacatctccttgcccctctagcttttcccatctcacagcctctggctttttcagtttaatttcaatctttgttgaaagtactttaaacgtgctctgttctggtattataggatgaagaagttccagtttcaaattgtaatcctctccagaaggaagtttaaccaaagcagacaactctttttctgaaaattccacatttacatcattcttctgaacattcttgatcataagtgtaatgactacttgagattctgtttgataccagtcatacttgatttttgactgatgagtccacacctcagattctgagccattctgagcttcttgacaccttttaatccagacactgaaattagcatctgcactatctaatttttgtccttctgtaaaagtttctagggcagcagcatagtttttttcatggtattcacatattccttttctcagcatagcagtggaattatttggattgagttctagagacttctttgcatcagcaacagcaacacagtaattcccaagaagaatgtgacaataagctctttgacaataatactgtgcatcatctggtttctgttccaaagccttagtcagctccggagctgagacgcagcatcaacaagagcctgggtccctgtccggcggtgcggggagaaggcgggtcagcggggacccgaagtggcccagctcccctaagaagagtggaggaagcagaaatgggctctctcacctctaacgccgcctgggggtcctcgtcgattagggcatccgagaagctctggaaaaacctctgggatgttgcagttcctgctgcagccgccgccatccctcgtagtcgctgttgctgccgccggagctgctactatcacggttaccacctccaccaccgcccaagggggaaacttctggagaaacaccaaccgagcttccgtcctaaatagccagcgagcagccacgcagcgtgctgctagggggacgggaggcgacacgccggcgcggggccggctgggacag

SEQ ID NO: 11167 - RNA, 3115 nt, Homo sapiens
  source 1..3115: mol_type = other RNA
ctgaatagctgggactacaggtgcatgccactacacccagctaatttttgcatttttagtagacacagggtttcaccatgttggccaggctggtcttgaactcctgacctcaggtgatctgcccacctccgcctcccaaaatgctgggattacaagcatgagctactgcacctggtcagaaacagctattttaatagtgtcatctttaagaaagaaaaagttaagcggcaaaaatatgcttctgtatttagaaccatggacctttaattataactctaagactctatggattatttacaaaggaactaagaaaggcctaaacctgctgaagattatgaaggtagtcaatgacagaagacttgctagagctaagcattcttgtctctggtatagtgctatacgtcctcaactatgcctctgcagcaatagccttcctcttcatcttaggattaatggtactgagaaaatttaacatacagaatacaaaagtcactatcctattttcctaagaagaaaactttagaaatccatccaaccaaaacttaattttgccttttccttcagtgttcaagaagaaaaaaatgtatctagtagctctaagtggacagaaggacaagtgaaaactctagaatgcttaaacaagctataacaacaggtttgggcaccatctggtatcaccttactgaaactttccttagtaactcccctacaccccacaacaaaggacgagaaggaaggagctgaattcctactgttttggaggctgaaatgatgacccgtttgcctcccactccccctgctctgagggtatagagtagtgctttgccataaaaatgttagtgacacctaacagagctgagaccaacatctggggtattacagttgagaaaatcatggtgagaaaacaaagtcagatctacaggtcatccatagtctatactttataacagcctagactgtaaacaattttaatcacagaacattttcctgtctctaaagtgtatttataccgagttcagcattcaatctttccacagttccttcatgaatgttattttttttccctgctacatttataagctctttgaagttaataatcatgtctttaattttttgtattctcatgatatctatatattctaggcacagagtaaatactaaacatatacacattaatttactctcacagcagttaccataaaccaatgaaaccaaagtaatcatggggacgtgacaacagagattttctaataaagaaaaaaaataccaaaaaacccaccaatgctgtaatttcaagaatcctgtcgtgataaaagaagcaagtggagttgggctttcctagaaccttctttgccctaccttcacagattatccttagtataaacttgcagtgtgttaaaactcaggtatctatgttttatacagaaacttgcaaggtaacgaccaaaatatctcagtgcaattaaatttacaaattcttcccattaaaagaactacatgggaattccctgtgataatttctcaaagttctcattaaaaacttaagaaaaaggtaaataaaccaaacatcttcatagaaaaattgtatttacaactccattcaaaagcagtttttaaaagcaaacacaatgtaacactgaaggtgaaaaatctaagctcacccaaagctgccaggtctaataaattactgacagaatactgtatcaaaaataaggcaataaccgaaaatataccattaaagatttctccatccccacaactagatagaatgaatctatctaggagcaaatgacatgctttattcagtttcaccatgtctgaaacctttaaggacagaagtgataaaatgttatcttcattcttcattagacttgaacacttgaaggaaaataatttctaaagcacaaagaggtaaagaagtataatctttcaaaaagatattcagtgttcaaaattcaagaatgcaatatcaatacacaatgggcattaggtgaatatacacaatacgatgagagcaaattaatttatttagtactttttccattccatatcatcaggaggattgatttcaactttccttttacctacatcagaccagttggtactcaaaactgtaccacccgactccataaaggatttgttcatggcacgtttcacttcatcagaaccatctgaatagatctgctgaaataatctgtttaaagctgcatctccctccaacttttcattcttttcttcttctttgatctcaccaaccaatttatcccaatttcttgtataaggagatgatgatggatataggttctttacatctgctacgaattgttttggcgtaggcacatctccttgcccctctagcttttcccatctcacagcctctggctttttcagtttaatttcaatctttgttgaaagtactttaaacgtgctctgttctggtattataggatgaagaagttccagtttcaaattgtaatcctctccagaaggaagtttaaccaaagcagacaactctttttctgaaaattccacatttacatcattcttctgaacattcttgatcataagtgtaatgactacttgagattctgtttgataccagtcatacttgatttttgactgatgagtccacacctcagattctgagccattctgagcttcttgacaccttttaatccagacactgaaattagcatctgcactatctaatttttgtccttctgtaaaagtttctagggcagcagcatagtttttttcatggtattcacatattccttttctcagcatagcagtggaattatttggattgagttctagagacttctttgcatcagcaacagcaacacagtaattcccaagaagaatgtgacaataagctctttgacaataatactgtgcatcatctggtttctgttccaaagccttagtcagctcctctaacgccgcctgggggtcctcgtcgattagggcatccgagaagctctggaaaaacctctgggatgttgcagttcctgctgcagccgccgccatccctcgtagtcgctgttgctgccgccggagctgctactatcacggttaccacctccaccaccgcccaagggggaaacttctggag

SEQ ID NO: 11168 - RNA, 3243 nt, Homo sapiens
  source 1..3243: mol_type = other RNA
ctgaatagctgggactacaggtgcatgccactacacccagctaatttttgcatttttagtagacacagggtttcaccatgttggccaggctggtcttgaactcctgacctcaggtgatctgcccacctccgcctcccaaaatgctgggattacaagcatgagctactgcacctggtcagaaacagctattttaatagtgtcatctttaagaaagaaaaagttaagcggcaaaaatatgcttctgtatttagaaccatggacctttaattataactctaagactctatggattatttacaaaggaactaagaaaggcctaaacctgctgaagattatgaaggtagtcaatgacagaagacttgctagagctaagcattcttgtctctggtatagtgctatacgtcctcaactatgcctctgcagcaatagccttcctcttcatcttaggattaatggtactgagaaaatttaacatacagaatacaaaagtcactatcctattttcctaagaagaaaactttagaaatccatccaaccaaaacttaattttgccttttccttcagtgttcaagaagaaaaaaatgtatctagtagctctaagtggacagaaggacaagtgaaaactctagaatgcttaaacaagctataacaacaggtttgggcaccatctggtatcaccttactgaaactttccttagtaactcccctacaccccacaacaaaggacgagaaggaaggagctgaattcctactgttttggaggctgaaatgatgacccgtttgcctcccactccccctgctctgagggtatagagtagtgctttgccataaaaatgttagtgacacctaacagagctgagaccaacatctggggtattacagttgagaaaatcatggtgagaaaacaaagtcagatctacaggtcatccatagtctatactttataacagcctagactgtaaacaattttaatcacagaacattttcctgtctctaaagtgtatttataccgagttcagcattcaatctttccacagttccttcatgaatgttattttttttccctgctacatttataagctctttgaagttaataatcatgtctttaattttttgtattctcatgatatctatatattctaggcacagagtaaatactaaacatatacacattaatttactctcacagcagttaccataaaccaatgaaaccaaagtaatcatggggacgtgacaacagagattttctaataaagaaaaaaaataccaaaaaacccaccaatgctgtaatttcaagaatcctgtcgtgataaaagaagcaagtggagttgggctttcctagaaccttctttgccctaccttcacagattatccttagtataaacttgcagtgtgttaaaactcaggtatctatgttttatacagaaacttgcaaggtaacgaccaaaatatctcagtgcaattaaatttacaaattcttcccattaaaagaactacatgggaattccctgtgataatttctcaaagttctcattaaaaacttaagaaaaaggtaaataaaccaaacatcttcatagaaaaattgtatttacaactccattcaaaagcagtttttaaaagcaaacacaatgtaacactgaaggtgaaaaatctaagctcacccaaagctgccaggtctaataaattactgacagaatactgtatcaaaaataaggcaataaccgaaaatataccattaaagatttctccatccccacaactagatagaatgaatctatctaggagcaaatgacatgctttattcagtttcaccatgtctgaaacctttaaggacagaagtgataaaatgttatcttcattcttcattagacttgaacacttgaaggaaaataatttctaaagcacaaagaggtaaagaagtataatctttcaaaaagatattcagtgttcaaaattcaagaatgcaatatcaatacacaatgggcattaggtgaatatacacaatacgatgagagcaaattaatttatttagtactttttccattccatatcatcaggaggattgatttcaactttccttttacctacatcagaccagttggtactcaaaactgtaccacccgactccataaaggatttgttcatggcacgtttcacttcatcagaaccatctgaatagatctgctgaaataatctgtttaaagctgcatctccctccaacttttcattcttttcttcttctttgatctcaccaaccaatttatcccaatttcttgtataaggagatgatgatggatataggttctttacatctgctacgaattgttttggcgtaggcacatctccttgcccctctagcttttcccatctcacagcctctggctttttcagtttaatttcaatctttgttgaaagtactttaaacgtgctctgttctggtattataggatgaagaagttccagtttcaaattgtaatcctctccagaaggaagtttaaccaaagcagacaactctttttctgaaaattccacatttacatcattcttctgaacattcttgatcataagtgtaatgactacttgagattctgtttgataccagtcatacttgatttttgactgatgagtccacacctcagattctgagccattctgagcttcttgacaccttttaatccagacactgaaattagcatctgcactatctaatttttgtccttctgtaaaagtttctagggcagcagcatagtttttttcatggtattcacatattccttttctcagcatagcagtggaattatttggattgagttctagagacttctttgcatcagcaacagcaacttccttttggcttaacatttagcttccttcttaaagctcttcaatgaatacagctgtgtcacaaaattcacctccttgtctcattaacattttctatgtaattttactcaaggtattcagtttttcccacagtaattcccaagaagaatgtgacaataagctctttgacaataatactgtgcatcatctggtttctgttccaaagccttagtcagctcctctaacgccgcctgggggtcctcgtcgattagggcatccgagaagctctggaaaaacctctgggatgttgcagttcctgctgcagccgccgccatccctcgtagtcgctgttgctgccgccggagctgctactatcacggttaccacctccaccaccgcccaagggggaaacttctggag

SEQ ID NO: 11169 - RNA, 1459 nt, Homo sapiens
  source 1..1459: mol_type = other RNA
ctgaatagctgggactacaggtgcatgccactacgcccggctaaatttttgtattttagtagagacggggtttcaccatgttgcccaggctggtctcgaactcctgaggtcaggcaatctgcccgccttggtcttccaaagtgctgggattagaggcatgagacactgtgcccagccaatttaaacattttctaattgacaaatggttgagttcacaattgtctgaagacctgggatcaataggaagcacatgttcaggttaagataaaagattataatacttcaaaaggttcttttgaagtcttataatggctacccttagagatgatagatgacaaatgtttcctattcagacctttaaaacaatgctagactctcagtctcttcaggattgggagggcctggaagaaaaagatctagctgtgttaatagagattctttacagatgcatattttcccccacaaagcacagctttgcaggaccatttcaaaatatggcaaagaaacatgttttggggtaaaatattttgactttcttctttgtcacatgtcatgccagagtcagactggaaagcaagtcaccatatatagggttaaataaaactcatctgatgagaatttatggtttgttgggcatgactccccaggccccttagataggaatttgggccagattaaaaaaaaaaaaaaaaatcaaagcttagtcctgaggcagcttctgaaatggtgggaaaaaatgtgagttttgaggaaacatttggttcagccattgttcttaagagatactgacatttcaacctactataaagagggaaatttaaagtattaaagtattaatgagttggtaggacccgcttttctttttttttttttttttaattcactggccccgaaagaaacttctctgtcaggccacaatataaccagataccagacacacgagatgttttggagggagggtggtggagccaagattgcagctccttattgaggaaaacagtcctcagagatccagagtcatttctcctgtgttcagcttgaaaaccttgggcaacttctggagatttcaacgtctcacagagtgcggaaacatgactggcgcagcatcctttccggaattggtgatgtccttcctgtaagggttgattttccatctcatcaaccaaatcgggaaagccgcagcatccttttctccaagaatgacaggtggtttatctcaggcttttctgtcccggcgcctttctctccaatgcagtctgctgatgtaatgcagtgattttttgtttgagggccacaggaagaccccttgtggctgttgtactggcattccctcttcatagcagggatggtgcctctggacattttccgacagcagggatcgttgggtgaggttagcagcgccagcccgggttagcggaagcagccttcaggtctcctaggagagcaggtttatgagcat

SEQ ID NO: 11170 - RNA, 12719 nt, Homo sapiens
  source 1..12719: mol_type = other RNA
ctgaatagctgggactacaggtgcatgccactatgcatgactaatttttgtatttttagtagagatggtgattttgtcatgttggccaggctggtctcgaactcctgacctcaagtcatccattcgccccggcctcccaaactgctggaattacaggctcacgccacttcatgaaatgtgttgtagtggctctggattctgtatcgttctgagaggtttttttcattggtttgttttcgtttttgtgtgtttccgtaggcaaaaaagttgcctggacaggtttacaaaacatatctccccatctccctgcagtcagcagctatcggtatctatgctaagttccttcaaagactcctaagaggtctccatggacctctgaagtttaatagtcaatgattgggtcagagcttactcagaaacctcaggccagtgaggcttccaacctctgcagcccaggctgagtggcttgagtagcacattcactgtgtggcagaactgcgagtctgcccaggcttttcatttcttctgggctccctggtgcctcccacgtgcatgtgtagaacagcattcagccagagatgcttgggaagtggatgagaacagcattcagccagagatgcttgggaagtggatgatgtctaccattctacggatcacttgcgatgcttatttcccagggaacagaaatgaagtggggccaggccatctcctgtctctgttgtctgtattacagaaggaagggagcggtgctggagcagggggcccaggagcatcacaggcggcaggccaaggagagagatgtaggtggcaggaccctccagggactcgggagagacacatgcgtgagcttttgcgatacggggtgagacagcaagggtgctgtggggtgtgtgtgccttcccccagacagtgtggatggctgcattcatgttagggctgtcataacaaagtaccgccagctgggagcgctatagaacgtcaatggattttctcacagttctggaaaccagaaattcaagatgaaggtgctgcagggttggcttccgccaaggcctctctccttggctcccagacggctgtcttctcccggcgtcctcacatgaaggtgcaaccccactatataacagtcagattggattaggacccaccctaatgtcctcattttaaccttacttaccttgtaaaggccctgtctccaaatacagccccattctggggtacggggtcggtgcagggtggggggtagggtttcaacatagagctttcaggagggcgcagttcagctagtgacagtgactgcaggtgtctaagcggagaggatgggccactccaacggggggcgggtgagcaaggggcgctggagaaagagcgtggagagcacgtgccgtctagtgtgcgcgctgggctggaaggtggggaccaggaggagaccgggaccacgagtaagagcccgcgagaggtacgtgtgagagcgactgtctccgtgtgggcgagaagcctggaaacggaggaactgggtttccgagggactgaatacctcggttgatagtctgcgcgctggcccagaaggaaggagcacaagcgcgcacgggatcccagcgtcttcccacaaccccgcctgcggctccgtccgctctccggcgccctctgctgggccagcagccgaaacgcaggggagcgctttccagcttcctccaatcccagcccacgcggtagccgctcacacgcaggtgcttaaacttaaatccatcaaaaattggcaagattaaaaaaatctcatgctggccacatttcaactgttctacgtggcatgtggctagtggcatcccttttgtacagcacagagaacatttccggcatctcagaaagttccatcagacgccctgctagtgaccaatctgcgaaaaagtgaggatcccaggctgcgcccagtggctcacgcctgtaatcccagtactttggggggccgaggcaggtggatcacctgaggtcaggagttccagaccagcctggccaacgtggtgaaaccccgtctctactaaaaatacaaaaattagctgggcgtggtggcgggcacctgtaatcccagctacttgagaggctgaagcaggagaatcgcttaaacccgggaggcagaggttgcagtgagccgaaatcacaccattgcactctagcctgggtgacgacagtgaaactccatctcaaattttaaaaaaaagtgagaatccccgactgtcccaaccacacacaacacacacacacacagcagctatctccttggttgagggcacttcccacttaggcccctccggacagtgttgtccaggacagaaacacacgtggccacacacacgccctcccctccatttatggctggcccagagctgcccagccagagagagaccacgcagggccaaaggaaataatctgctatcaaaactgaaagaggccaggtgcggtggctcacggctgtaatcccagcactttgggaggccgaggtgggcggaatcacaaggtcagattgagaccatcctggctaacacggtgaaaccccgtctctactaacaatacaaaaaattagcttagccgggcgtggtggtgggcgcctgtagtcccagctactcgggaggctgaggcaggagaatggcatgaacccgggaggtggagcttgcagtgagccgagatcgcaccactgcactccagcctgggtgacagtgcaagactccgtctcaaaaaaaaaacaacagtgaaagaaaagaaaggagtaaatgcggcttagatgaacgaataaatgcattcacccattctacctgaaatcaatacccaattgatgtaagaaacagaaatcatttaggtagatagggcgaagagagtccccagcaaaaaacttcctaacaaaaagcagcttagaaattgctccctttctcaccacaccacgcagttcaaagaaatcacttctcctaacaaagagcagcctgatctttcaggctgtaaaacacagataagcaactcgggcacagacttgggaggttcctgggtaatcaccaagccacatacatagatgggccccagtgaaaacagtgggcctaaagcacattcctttccctttctttaggcacactaagggaagctggaagcgcgtgggggagatgcctgcagctgcacgaaggtgcctgggaatgggcacagaaacactccctccccttttagcacacacagataagcagcagcgcagagcagcacaaacgaagggcctgcctgcaggatcaaagaatggggtgggggcccggcgcggtggctcacgcctgcaatcccactactttgggaggccgaggcaggcggatcacttgaggtcaggagttggagaccagcctgaccaacatggtgaaaccttgtctctactaaaaatacaaaattagccgggcatggctgcatgcacctgtaatcccgactacgcgggaggctgaggcacgagaattgcttgaacctgggaggcggaggttgcagtgagccaagatgacaccactgcactccagcctgggcgacagagcgagactccatctcaaaaaaaaaaaaaaaaaaaagaatggggtgggggctgctagagactctgctcgatgcagacagcacacctggtcctaactggttcttcaggccctaggaagaaaagacacccctcctcactagcccatctataaaacccctgacatttcttctacaacttcacaacccgttcgggacccgtctctgtgacagagctgtttcttccttttgcctattaaactcctgctccaaatctcactctgtgtgcatccacatccttgatttcctcggctgtgagaccaaaaaccttagtatttaccacagacaagaccgttttacaggaacaagccaggcagggtcccgaaagctcagtattttaagggtctaacagggagaagttctcattaatgtcagctccttctgagaactgctggggtcagaatagtccgggaaaggggagaggagacacaaggtccttgttcaaatcatgtatttcttaagatactaagagaaaaaaatacaggaaacagtatcattttttttttttttttggagacagggtctcactctgtcacccaggctggagtgcagtagtgcaatctcggctcactacaacctccgcctcctgggttcaagcgattctcctgcctcagcctcctaagtagctgggattacaggtgcccgccaccacactaggctaatttttgtatttttagtagagacggggtttcgccatgttggccaggctggtctcgaactcctgacctcgtgatccgcccgcctcggcctcccaaagtgctaggattacaagcatgagccacagcacccaggcgaaacagtatcatttctaacccttttcatgtggctgtcaggacatgtttcaagcaccgagtccagcatcttgataagatgggaaccagggagccctcagggcccccgcgccagccctcccactgcaaacccacaccaccctggccgtctggagcttgtcccagcccggctccccgtgacatcgggacctggccactcctggacgtgatgccctaagcttgcctcccctgcggatggatgtagtgatgcttgatttgggtggatgagaacattccccacaacacaagccattttgcaacctcacctcccgagcctctgagctacctttcattcccctctgagcacgcagggttaactgctgtaggggttacccccatcaatgcatgagttataccttttgacagtaacacacaacgattactagagagcatgtcattaccatttttaagtgctccaggggaggggccatgaggaggctgtaggtgaaacaggagtggttcaaatgtaaatgatggctgaacacgagtgaggcatttgcaggggtggttatgataatattgtctatagttttgtgtgcttcaagatgtccctcagaaagtttgtaattatgggccgggtgccgtggctcacgcctgtaatcccagcactttgggaggccgaggcgggtggatcacaaggtcaggagttcgaccagcctggccaatatggtgaaaccctgtctctgctaaaaacagaaaaatgagttggctgtggtcgcacgcacctgtagtcccaagtcaggagaatcgcttgaacccgggaggcggaggttgcagtgagccgagatcgcgccactgcactccagcctgggggacgagagcaagactccatctcaaaaaaaaaataaataataataataaggaaaggaagtttgtatttatggagcagtcattaaatagtgctttatgggccgggcacagtggctcaagcctgtaatcccaacactttggaaggccgaggtgggcagatcacgaggtcaggagatcgtgaccatcctggctaacacagtgaaaccccgtctctactaaaaaaatacaaaaaaattagctgggcatggtggtgggcatctgtagtcccagctacttgggaggctgaggcaggagaatggcgtgaacacaggaggcggagcttgcagtgagcagagatcgagccactgcactccagcctgggcgacagagcaagactctgtctcaaaaaaaaaaaatagtgctttaggaaattataaatatccatactaaaataatgtggatgaaacataacattatataattatccctgaaagtaaaacaaaagcatgaagaaacattcaatacaaaacaaacagcaaagggagcgatttctcggcggaaagcatgctggaaccctgtggaagcgtgggctgtcccaggacgtgcaggcaggccttagacccctgccacatacaagcaatcaccgggggtcagcacactttttgttgaagagccagatagtaaatattttaggctcaagggacactcggtctctgccacactcaatgtcaccattgccactgtagtgcagaagcagccgtggctgcactctaataaaacatttttttttacaaaagcaagcagccaatccttgggctgcagtttgagaaactccaggggcacctgtgatgtgagtaggccggtttctcaccacagtgaagggcctggcaggatggcgcttgagggatgagctggacaacccacagtcatcacagagacagacaagttctcaagaaataaaacatttctggccggacgcaatggctcacgccacacccgggaagctagaagcacgtgtgggggagatgcctgcggctgcaagaaggtgcctgggaatgggcacagaaactctccctccccttttagcacacgcagaaaaccaacgcagagcagcacaaactaagggcctgggggaggcgggagggaaggcattaggagatatacctaatgtaaatgacgagttaatgcgtgcagcacaccaacatggcacatgtatatatatgtaacaaacctgcgcgttgtgcataggtaccctagaacttaaagtataataaaaaaataaaaaatgaaatggggtgggggccgctacagtggctcacgcctgtaatcccagcactttgggaggccgaggcaggcggatcacgaggtcaggagatcgagaccatcctaacatggtgaaaccccgtctgtactaaaaatacaaaaaaaaattagctgggcgtggtggtgggcacctgtaatcccagctactcgagaggctgaggcaggagaatcgcttgaacccgggaggtggaggttgcggtgagccgagatcgtgccactgcactccagcctggcaacagagcaagactccttctaggggggaaaaaaaagggcatttcttcctattcaatgagaacatgaggaaaaggcaaaaggcagaggctggctgggagtgggtttgtgtgtgtaaaattgagtttcagtataaaaaaagatcaaggcaggactgaaagccctgaggctggcatcgcagctccagagcgaggggcaagcgtagggcgaggagcgaggatagggcgagggcgggagtagagcgaggggtaaggctagggtgagcacaggtggcaggggactctggtgggcctggactctggtgggcggggtgacccaggagctcggatgaagctcctacgggctccaggaaggttccctcaagtgccttccccacccaacccctaggccctgaacagagtcgagacccaggaatgtcccacgccccatcgcttcacctgtcccagggagaaattctggggttttttccacttcagccctctctgggggaagacgtcgggtcagaagcacatctgctcctgagagccagccgggagcaccaccatgactcttgcttagccaaacctgagggatctgaacctcctcctaggcccatccgtgcatgcccttgtaaaatcctttcagcaaatgaaccccgccgccatcccccccaacccccgccaccctcacatctgataggcttcttcagcctccaccatccccaggtgacctctgatcaccctggcctgccttcagcaagaatcctgctaggtgggtttagccgaaaacccccggacccctgaggtttgctcttagtgattttccatccactgatggtacctgtacctgtctcgatggtcctgaataaagtcttcctcacggccatttaacaagctcgccatcccactgtggggagagagacacatctgctgtagaaagagtgatacacacacagtggggggagccctcaatcggggacaacagcaggctcccagcattctcccagcgttcaaccgtgtatgtcactaagctcaggtgcttgggcctcatgggggactcctacacagcagctcctgctgagcactttggtggctggaatattctagaaagaggaataaagtaggagacacgagatctgtggtgctactttgtaattcgcactgtagggaaaagaagatgccgaagatgctgtagttaagccccaaatttatgtgcaagcctctgggtttttgtcttgtttttcaatcctgtcttctctgttttgccaaatgaggaaatggtggggagaattaaagcctcacacctttaacccctccactggactaatccaactgtatcattttatcttcgtcctcagcttttttgaagagaaagggagtgcaggctccgcagtgcgaaatcgtgaaacttatccttaatttggtgaatggagggtctgacaagtgaggggcccaggagctatgaccctgtggggagaccaagattggcaagagggaggctcggctcgcctcccctttccatgtgatcccacccagagctgccgccttcagctggctctctgtgccctgtggggctcccccatcacaaccgcctagagcagcagggtctcggacagcccaagcgtaagggacgcttgctgctgcctggggacagcaccccctcccccggtaacagtccccatttcctcctgggaaatgactctcccacaacatacccaggccgggtgtgagaagagggcttcccctccctggctaagcaagggggatgctcctctgcaactgaatctggaaccggctgaccccaaagttcctgtgtccctgggacccacctcttcctgcatggtgtggtcagcaattcctccatcaagcccccgacaaccctccagacaccctggtctgcaggggcaagtggaggccagagaacgctccgacacaggtcatgacccaattcacagcaagaaacagaaccccaacctcacatcaccccaacagcactccttttgctctgcaatccccaggtgacgtaggtctgtccaccagggagtgggcacacagggtggccacgacgctgctcggacaccgcagtcatgtccctctcagtggcctccaacactccactggctgggtgctccctggaccccgacccataacaagtgtccctgtgatgtagctgtctggccccaccctgagcccagagcgtcccccgggcagaaggggcaagaagtctgaccccaggggcctggccccacacagccttcaccccagcacctctgagacaagagctgtcggagtcactgagggagcgaacccagccgtcaggacttgaccccaggggatcacggagggagactccacatggaagaacagcctgttcggcttaaaacagacatggccagatccccatccctgaggccctggctgtggggcctgcaacaagctgtcacctagccctggagatgacagcaacacccccctcacaaggcggcccgaggattctcccggatagtctcaccaggtgtggtccagcccaggacaagagcacacagaggaaaacagcacacagaggacaaccaggaggcgcctggtggtccactcagctcagccggcagaggctgacccggctttccaggagtgcagggatggattagtgatgcttgcggtgggcccgggcgatggcgacggtgacctgtgttgcacatgtgccatctctcaggattcttctcctccctgaaccccagtgcactctctgacctcatcctggtgtcccctcaacacaagagcaaggcctcctgcaccggaagcgtctggccatgagtggcctcccgaccacctggacctgtgtgggctacagctccgccaggcctcgcacagtccaccctcaacccagccatcccttgacctgggagggtcagggaaatcagggcttctgagacagaggggctggttgccagccacccccgagaaagagatgtgacctgagccctgggtccctggatgaaggggctctgggggacacacgaaatcacagatgggaatctgggagtgccaagcccgtgggaattgccatttattcccaaagttgccaaaatcatcaccaaggattcaccgagggtgcgtgagcgggtgcgtgaggggaacgaggaggctcaaacactgactgggggttgggagtttggagggagggggaatgggtgggggccccagccacccctcccccttctaatgccacgggaaaggggtcctcctctggccagctcccctccccaggccccatgtccagtttctctccggggaggtggggtgggaaaggaagagggtgtagtgtgagtgggccccaggaaggggaagggcactgggggtggggatcccccatttcacatgcactcacaacactgatctcccagggagccggaatggggcagccggatggagccaggcccccttccgccctggattataggaggaagggattagtgttgggggccggggggcccgggggcatcatggggggcaggccagggcccccgccaaggggagagatgtacgtgggtggcgctccagggacgggaggcacaggactgagacggagctggttcagggtgagcgtcgcgggaggcgcgggctggaaggggttggtgacggaagggccagtggctgggcctccgcctggcaggaaggggttggaggccttggctccaggcggcgtggggcccggccggctcaccagcgagtccaggtcgacgagggctgcattgggccccaggaatgactccggcgtcttccgggtggggggcgtgggagttggtgtggctgcaggtggggggctgcccacagcctcagccagagatcccctgaccccactcatgtcaaacgccccagggcttcgggccggcacctctcctgccagcagctccagctctcctgcgctgctcccggaggtcggcagtgccgtgcggagtcggtcaaagtcagagaactcgtcgggctccgtgtcgaatcccccggctgctgttgtgccattggtgctgggcttggcaggtgaccctccccagggatctgagaaggccggggccggtgtccagggatcggaggctgagggcccactgaccgggaccccaccatcggaacttccccatggatcaggcgtgggcccctccccagctgcaggggctggggtcccaccccaagggtcaactgagggtcctgcaggggcagcaggcctccaggggtccccagaggccggcgtgggggctggacctccccagggatcagcagctggagggacaggggggccgccccaggggtccgaggtgggggcagccgtggggacggcagcagccatgggtgctgggcccccccaggggtctgtggtcggggcaggagctggggccgtgaagacgtcagcaaggtccatgagggacgactcctccttgcccccagtctccctcttgctctcctcgattgccatctgcagccgcaggtcatccccgcgacggatccgctcctcctggtcggcctcctccttgctcatggccagggccagctggagctgcagctcctcctccccgctgctctgcggccacgcctgctccgcctcgggaggggggcctgagcccacagctgctgatgaggccgtggcggtctgtgccagcttttccttggtcttgagcgcgtgcgcccgctcttcccgcagccggtcctcgtcgcgcagcagggccaccagctgcttagctttctcacgcacgttcacgccctggtccttgccgtcgcggtccacgtactggaagtccttcagcgtctgcacggcgtacatgttctccttgcactgctgcgacacgcgctccgagccggtcttgatgaggtactccatcagcgtcatggccttgtaaacgtgacgccagttcttgccatggtcattgagccgcttccagatcatgctcatgatctccgagaaggcgacaacgttgtaggtgaggtcggcaatctctgacatgagggagctggatgggccccaggggtcattgctcgtggcctctcgaaccttgatctccgcctctgagtagttgtggacgatgttcttcatctggcgcctcaaggacgaggtcgacatggtgcccggctgcagcagcaaggggcacagggccccgatgcgtggagagatggggcgactcccggacgaaggctgcggcaggtgctggcaggtcaccgcatccagggcggcaggaagaaccggggaagccagaagaccagacgtcccaaggatagcggaagcccaaggctcaggagagataaggaacctaacagccccactgcctgggtccctgctgtgtgccaggtgctcgctcagcacaagagggacattacctttttcaacactgcatgcaaagactgggctccttactcctggagcagcctggttccagagccagctctgatcacccatctatgcggctccaagaagccacagagggagattttcaaagccccgccatgatgtaagcccaggggagatagggatgacggagagaggctggcctctgcttccacctcaggccagaaagccaggcacctgaagacagatgtagctagttaaaaagtaactctctggagtcccaaaacagccccagcctaatacattaagatgaagagatgatgtaacaaatgcagagaaggggactgagaagaaatagaagacagttctgacagaaagagacacatagaaacctgggcagagggagctaggcagagacacaatgagaaaaacacaggcagcagcagatacaagaacatgggaagacagggaggcaggaggccaaggaagaaagaggcccagaaacaaaaagagacctggcgctgagaaataagagataagaaaaatggaatctaatggcaaagaatataaaatgtgggttcaaatcctggccacatcagctacctgcagcgcacacctccttgagacacagtttgctcaactctgaaatgaaag

SEQ ID NO: 11171 - RNA, 12229 nt, Homo sapiens
  source 1..12229: mol_type = other RNA
ctgaatagctgggactacaggtgcatgccactatgcatgactaatttttgtatttttagtagagatggtgattttgtcatgttggccaggctggtctcgaactcctgacctcaagtcatccattcgccccggcctcccaaactgctggaattacaggctcacgccacttcatgaaatgtgttgtagtggctctggattctgtatcgttctgagaggtttttttcattggtttgttttcgtttttgtgtgtttccgtaggcaaaaaagttgcctggacaggtttacaaaacatatctccccatctccctgcagtcagcagctatcggtatctatgctaagttccttcaaagactcctaagaggtctccatggacctctgaagtttaatagtcaatgattgggtcagagcttactcagaaacctcaggccagtgaggcttccaacctctgcagcccaggctgagtggcttgagtagcacattcactgtgtggcagaactgcgagtctgcccaggcttttcatttcttctgggctccctggtgcctcccacgtgcatgtgtagaacagcattcagccagagatgcttgggaagtggatgagaacagcattcagccagagatgcttgggaagtggatgatgtctaccattctacggatcacttgcgatgcttatttcccagggaacagaaatgaagtggggccaggccatctcctgtctctgttgtctgtattacagaaggaagggagcggtgctggagcagggggcccaggagcatcacaggcggcaggccaaggagagagatgtaggtggcaggaccctccagggactcgggagagacacatgcgtgagcttttgcgatacggggtgagacagcaagggtgctgtggggtgtgtgtgccttcccccagacagtgtggatggctgcattcatgttagggctgtcataacaaagtaccgccagctgggagcgctatagaacgtcaatggattttctcacagttctggaaaccagaaattcaagatgaaggtgctgcagggttggcttccgccaaggcctctctccttggctcccagacggctgtcttctcccggcgtcctcacatgaaggtgcaaccccactatataacagtcagattggattaggacccaccctaatgtcctcattttaaccttacttaccttgtaaaggccctgtctccaaatacagccccattctggggtacggggtcggtgcagggtggggggtagggtttcaacatagagctttcaggagggcgcagttcagctagtgacagtgactgcaggtgtctaagcggagaggatgggccactccaacggggggcgggtgagcaaggggcgctggagaaagagcgtggagagcacgtgccgtctagtgtgcgcgctgggctggaaggtggggaccaggaggagaccgggaccacgagtaagagcccgcgagaggtacgtgtgagagcgactgtctccgtgtgggcgagaagcctggaaacggaggaactgggtttccgagggactgaatacctcggttgatagtctgcgcgctggcccagaaggaaggagcacaagcgcgcacgggatcccagcgtcttcccacaaccccgcctgcggctccgtccgctctccggcgccctctgctgggccagcagccgaaacgcaggggagcgctttccagcttcctccaatcccagcccacgcggtagccgctcacacgcaggtgcttaaacttaaatccatcaaaaattggcaagattaaaaaaatctcatgctggccacatttcaactgttctacgtggcatgtggctagtggcatcccttttgtacagcacagagaacatttccggcatctcagaaagttccatcagacgccctgctagtgaccaatctgcgaaaaagtgaggatcccaggctgcgcccagtggctcacgcctgtaatcccagtactttggggggccgaggcaggtggatcacctgaggtcaggagttccagaccagcctggccaacgtggtgaaaccccgtctctactaaaaatacaaaaattagctgggcgtggtggcgggcacctgtaatcccagctacttgagaggctgaagcaggagaatcgcttaaacccgggaggcagaggttgcagtgagccgaaatcacaccattgcactctagcctgggtgacgacagtgaaactccatctcaaattttaaaaaaaagtgagaatccccgactgtcccaaccacacacaacacacacacacacagcagctatctccttggttgagggcacttcccacttaggcccctccggacagtgttgtccaggacagaaacacacgtggccacacacacgccctcccctccatttatggctggcccagagctgcccagccagagagagaccacgcagggccaaaggaaataatctgctatcaaaactgaaagaggccaggtgcggtggctcacggctgtaatcccagcactttgggaggccgaggtgggcggaatcacaaggtcagattgagaccatcctggctaacacggtgaaaccccgtctctactaacaatacaaaaaattagcttagccgggcgtggtggtgggcgcctgtagtcccagctactcgggaggctgaggcaggagaatggcatgaacccgggaggtggagcttgcagtgagccgagatcgcaccactgcactccagcctgggtgacagtgcaagactccgtctcaaaaaaaaaacaacagtgaaagaaaagaaaggagtaaatgcggcttagatgaacgaataaatgcattcacccattctacctgaaatcaatacccaattgatgtaagaaacagaaatcatttaggtagatagggcgaagagagtccccagcaaaaaacttcctaacaaaaagcagcttagaaattgctccctttctcaccacaccacgcagttcaaagaaatcacttctcctaacaaagagcagcctgatctttcaggctgtaaaacacagataagcaactcgggcacagacttgggaggttcctgggtaatcaccaagccacatacatagatgggccccagtgaaaacagtgggcctaaagcacattcctttccctttctttaggcacactaagggaagctggaagcgcgtgggggagatgcctgcagctgcacgaaggtgcctgggaatgggcacagaaacactccctccccttttagcacacacagataagcagcagcgcagagcagcacaaacgaagggcctgcctgcaggatcaaagaatggggtgggggcccggcgcggtggctcacgcctgcaatcccactactttgggaggccgaggcaggcggatcacttgaggtcaggagttggagaccagcctgaccaacatggtgaaaccttgtctctactaaaaatacaaaattagccgggcatggctgcatgcacctgtaatcccgactacgcgggaggctgaggcacgagaattgcttgaacctgggaggcggaggttgcagtgagccaagatgacaccactgcactccagcctgggcgacagagcgagactccatctcaaaaaaaaaaaaaaaaaaaagaatggggtgggggctgctagagactctgctcgatgcagacagcacacctggtcctaactggttcttcaggccctaggaagaaaagacacccctcctcactagcccatctataaaacccctgacatttcttctacaacttcacaacccgttcgggacccgtctctgtgacagagctgtttcttccttttgcctattaaactcctgctccaaatctcactctgtgtgcatccacatccttgatttcctcggctgtgagaccaaaaaccttagtatttaccacagacaagaccgttttacaggaacaagccaggcagggtcccgaaagctcagtattttaagggtctaacagggagaagttctcattaatgtcagctccttctgagaactgctggggtcagaatagtccgggaaaggggagaggagacacaaggtccttgttcaaatcatgtatttcttaagatactaagagaaaaaaatacaggaaacagtatcattttttttttttttttggagacagggtctcactctgtcacccaggctggagtgcagtagtgcaatctcggctcactacaacctccgcctcctgggttcaagcgattctcctgcctcagcctcctaagtagctgggattacaggtgcccgccaccacactaggctaatttttgtatttttagtagagacggggtttcgccatgttggccaggctggtctcgaactcctgacctcgtgatccgcccgcctcggcctcccaaagtgctaggattacaagcatgagccacagcacccaggcgaaacagtatcatttctaacccttttcatgtggctgtcaggacatgtttcaagcaccgagtccagcatcttgataagatgggaaccagggagccctcagggcccccgcgccagccctcccactgcaaacccacaccaccctggccgtctggagcttgtcccagcccggctccccgtgacatcgggacctggccactcctggacgtgatgccctaagcttgcctcccctgcggatggatgtagtgatgcttgatttgggtggatgagaacattccccacaacacaagccattttgcaacctcacctcccgagcctctgagctacctttcattcccctctgagcacgcagggttaactgctgtaggggttacccccatcaatgcatgagttataccttttgacagtaacacacaacgattactagagagcatgtcattaccatttttaagtgctccaggggaggggccatgaggaggctgtaggtgaaacaggagtggttcaaatgtaaatgatggctgaacacgagtgaggcatttgcaggggtggttatgataatattgtctatagttttgtgtgcttcaagatgtccctcagaaagtttgtaattatgggccgggtgccgtggctcacgcctgtaatcccagcactttgggaggccgaggcgggtggatcacaaggtcaggagttcgaccagcctggccaatatggtgaaaccctgtctctgctaaaaacagaaaaatgagttggctgtggtcgcacgcacctgtagtcccaagtcaggagaatcgcttgaacccgggaggcggaggttgcagtgagccgagatcgcgccactgcactccagcctgggggacgagagcaagactccatctcaaaaaaaaaataaataataataataaggaaaggaagtttgtatttatggagcagtcattaaatagtgctttatgggccgggcacagtggctcaagcctgtaatcccaacactttggaaggccgaggtgggcagatcacgaggtcaggagatcgtgaccatcctggctaacacagtgaaaccccgtctctactaaaaaaatacaaaaaaattagctgggcatggtggtgggcatctgtagtcccagctacttgggaggctgaggcaggagaatggcgtgaacacaggaggcggagcttgcagtgagcagagatcgagccactgcactccagcctgggcgacagagcaagactctgtctcaaaaaaaaaaaatagtgctttaggaaattataaatatccatactaaaataatgtggatgaaacataacattatataattatccctgaaagtaaaacaaaagcatgaagaaacattcaatacaaaacaaacagcaaagggagcgatttctcggcggaaagcatgctggaaccctgtggaagcgtgggctgtcccaggacgtgcaggcaggccttagacccctgccacatacaagcaatcaccgggggtcagcacactttttgttgaagagccagatagtaaatattttaggctcaagggacactcggtctctgccacactcaatgtcaccattgccactgtagtgcagaagcagccgtggctgcactctaataaaacatttttttttacaaaagcaagcagccaatccttgggctgcagtttgagaaactccaggggcacctgtgatgtgagtaggccggtttctcaccacagtgaagggcctggcaggatggcgcttgagggatgagctggacaacccacagtcatcacagagacagacaagttctcaagaaataaaacatttctggccggacgcaatggctcacgccacacccgggaagctagaagcacgtgtgggggagatgcctgcggctgcaagaaggtgcctgggaatgggcacagaaactctccctccccttttagcacacgcagaaaaccaacgcagagcagcacaaactaagggcctgggggaggcgggagggaaggcattaggagatatacctaatgtaaatgacgagttaatgcgtgcagcacaccaacatggcacatgtatatatatgtaacaaacctgcgcgttgtgcataggtaccctagaacttaaagtataataaaaaaataaaaaatgaaatggggtgggggccgctacagtggctcacgcctgtaatcccagcactttgggaggccgaggcaggcggatcacgaggtcaggagatcgagaccatcctaacatggtgaaaccccgtctgtactaaaaatacaaaaaaaaattagctgggcgtggtggtgggcacctgtaatcccagctactcgagaggctgaggcaggagaatcgcttgaacccgggaggtggaggttgcggtgagccgagatcgtgccactgcactccagcctggcaacagagcaagactccttctaggggggaaaaaaaagggcatttcttcctattcaatgagaacatgaggaaaaggcaaaaggcagaggctggctgggagtgggtttgtgtgtgtaaaattgagtttcagtataaaaaaagatcaaggcaggactgaaagccctgaggctggcatcgcagctccagagcgaggggcaagcgtagggcgaggagcgaggatagggcgagggcgggagtagagcgaggggtaaggctagggtgagcacaggtggcaggggactctggtgggcctggactctggtgggcggggtgacccaggagctcggatgaagctcctacgggctccaggaaggttccctcaagtgccttccccacccaacccctaggccctgaacagagtcgagacccaggaatgtcccacgccccatcgcttcacctgtcccagggagaaattctggggttttttccacttcagccctctctgggggaagacgtcgggtcagaagcacatctgctcctgagagccagccgggagcaccaccatgactcttgcttagccaaacctgagggatctgaacctcctcctaggcccatccgtgcatgcccttgtaaaatcctttcagcaaatgaaccccgccgccatcccccccaacccccgccaccctcacatctgataggcttcttcagcctccaccatccccaggtgacctctgatcaccctggcctgccttcagcaagaatcctgctaggtgggtttagccgaaaacccccggacccctgaggtttgctcttagtgattttccatccactgatggtacctgtacctgtctcgatggtcctgaataaagtcttcctcacggccatttaacaagctcgccatcccactgtggggagagagacacatctgctgtagaaagagtgatacacacacagtggggggagccctcaatcggggacaacagcaggctcccagcattctcccagcgttcaaccgtgtatgtcactaagctcaggtgcttgggcctcatgggggactcctacacagcagctcctgctgagcactttggtggctggaatattctagaaagaggaataaagtaggagacacgagatctgtggtgctactttgtaattcgcactgtagggaaaagaagatgccgaagatgctgtagttaagccccaaatttatgtgcaagcctctgggtttttgtcttgtttttcaatcctgtcttctctgttttgccaaatgaggaaatggtggggagaattaaagcctcacacctttaacccctccactggactaatccaactgtatcattttatcttcgtcctcagcttttttgaagagaaagggagtgcaggctccgcagtgcgaaatcgtgaaacttatccttaatttggtgaatggagggtctgacaagtgaggggcccaggagctatgaccctgtggggagaccaagattggcaagagggaggctcggctcgcctcccctttccatgtgatcccacccagagctgccgccttcagctggctctctgtgccctgtggggctcccccatcacaaccgcctagagcagcagggtctcggacagcccaagcgtaagggacgcttgctgctgcctggggacagcaccccctcccccggtaacagtccccatttcctcctgggaaatgactctcccacaacatacccaggccgggtgtgagaagagggcttcccctccctggctaagcaagggggatgctcctctgcaactgaatctggaaccggctgaccccaaagttcctgtgtccctgggacccacctcttcctgcatggtgtggtcagcaattcctccatcaagcccccgacaaccctccagacaccctggtctgcaggggcaagtggaggccagagaacgctccgacacaggtcatgacccaattcacagcaagaaacagaaccccaacctcacatcaccccaacagcactccttttgctctgcaatccccaggtgacgtaggtctgtccaccagggagtgggcacacagggtggccacgacgctgctcggacaccgcagtcatgtccctctcagtggcctccaacactccactggctgggtgctccctggaccccgacccataacaagtgtccctgtgatgtagctgtctggccccaccctgagcccagagcgtcccccgggcagaaggggcaagaagtctgaccccaggggcctggccccacacagccttcaccccagcacctctgagacaagagctgtcggagtcactgagggagcgaacccagccgtcaggacttgaccccaggggatcacggagggagactccacatggaagaacagcctgttcggcttaaaacagacatggccagatccccatccctgaggccctggctgtggggcctgcaacaagctgtcacctagccctggagatgacagcaacacccccctcacaaggcggcccgaggattctcccggatagtctcaccaggtgtggtccagcccaggacaagagcacacagaggaaaacagcacacagaggacaaccaggaggcgcctggtggtccactcagctcagccggcagaggctgacccggctttccaggagtgcagggatggattagtgatgcttgcggtgggcccgggcgatggcgacggtgacctgtgttgcacatgtgccatctctcaggattcttctcctccctgaaccccagtgcactctctgacctcatcctggtgtcccctcaacacaagagcaaggcctcctgcaccggaagcgtctggccatgagtggcctcccgaccacctggacctgtgtgggctacagctccgccaggcctcgcacagtccaccctcaacccagccatcccttgacctgggagggtcagggaaatcagggcttctgagacagaggggctggttgccagccacccccgagaaagagatgtgacctgagccctgggtccctggatgaaggggctctgggggacacacgaaatcacagatgggaatctgggagtgccaagcccgtgggaattgccatttattcccaaagttgccaaaatcatcaccaaggattcaccgagggtgcgtgagcgggtgcgtgaggggaacgaggaggctcaaacactgactgggggttgggagtttggagggagggggaatgggtgggggccccagccacccctcccccttctaatgccacgggaaaggggtcctcctctggccagctcccctccccaggccccatgtccagtttctctccggggaggtggggtgggaaaggaagagggtgtagtgtgagtgggccccaggaaggggaagggcactgggggtggggatcccccatttcacatgcactcacaacactgatctcccagggagccggaatggggcagccggatggagccaggcccccttccgccctggattataggaggaagggattagtgttgggggccggggggcccgggggcatcatggggggcaggccagggcccccgccaaggggagagatgtacgtgggtggcgctccagggacgggaggcacaggactgagacggagctggttcagggtgagcgtcgcgggaggcgcgggctggaaggggttggtgacggaagggccagtggctgggcctccgcctggcaggaaggggttggaggccttggctccaggcggcgtggggcccggccggctcaccagcgagtccaggtcgacgagggctgcattgggccccaggaatgactccggcgtcttccgggtggggggcgtgggagttggtgtggctgcaggtggggggctgcccacagcctcagccagagatcccctgaccccactcatgtcaaacgccccagggcttcgggccggcacctctcctgccagcagctccagctctcctgcgctgctcccggaggtcggcagtgccgtgcggagtcggtcaaagtcagagaactcgtcgggctccgtgtcgaatcccccggctgctgttgtgccattggtgctgggcttggcaggtgaccctccccagggatctgagaaggccggggccggtgtccagggatcggaggctgagggcccactgaccgggaccccaccatcggaacttccccatggatcaggcgtgggcccctccccagctgcaggggctggggtcccaccccaagggtcaactgagggtcctgcaggggcagcaggcctccaggggtccccagaggccggcgtgggggctggacctccccagggatcagcagctggagggacaggggggccgccccaggggtccgaggtgggggcagccgtggggacggcagcagccatgggtgctgggcccccccaggggtctgtggtcggggcaggagctggggccgtgaagacgtcagcaaggtccatgagggacgactcctccttgcccccagtctccctcttgctctcctcgattgccatctgcagccgcaggtcatccccgcgacggatccgctcctccttatcatgctcttctcggctcaaactaagggccagctggagctgggcgtcgtcctcggggccgcaggacgggggctggtcggcctcctccttgctcatggccagggccagctggagctgcagctcctcctccccgctgctctgcggccacgcctgctccgcctcgggaggggggcctgagcccacagctgctgatgaggccgtggcggtctgtgccagcttttccttggtcttgagcgcgtgcgcccgctcttcccgcagccggtcctcgtcgcgcagcagggccaccagctgcttagctttctcacgcacgttcacgccctggtccttgccgtcgcggtccacgtactggaagtccttcagcgtctgcacggcgtacatgttctccttgcactgctgcgacacgcgctccgagccggtcttgatgaggtactccatcagcgtcatggccttgtaaacgtgacgccagttcttgccatggtcattgagccgcttccagatcatgctcatgatctccgagaaggcgacaacgttgtaggtgaggtcggcaatctctgacatgagggagctggatgggccccaggggtcattgctcgtggcctctcgaaccttgatctccgcctctgagtagttgtggacgatgttcttcatctggcgcctcaaggacgaggtcgacatggtgcccggctgcagcagcaaggggcacagggccccgatgcgtggagagatggggcgactcccggacgaaggctgcggcaggtgctggcaggtcaccgcatctcggccccctcacgccgggctctggggggtcatggcggtcagccccctgccccgctcggcctcggtgtcgcgggacgtgcgccgggccacgggcgcacgcacgaacgcaaggagggccgcacgccgacggctccgccgccccgccgcccagaaggggcgcggagagccgggcgggggaggggagccgccgaggagacgggaagcaacag

SEQ ID NO: 11172 - RNA, 12151 nt, Homo sapiens
  source 1..12151: mol_type = other RNA
ctgaatagctgggactacaggtgcatgccactatgcatgactaatttttgtatttttagtagagatggtgattttgtcatgttggccaggctggtctcgaactcctgacctcaagtcatccattcgccccggcctcccaaactgctggaattacaggctcacgccacttcatgaaatgtgttgtagtggctctggattctgtatcgttctgagaggtttttttcattggtttgttttcgtttttgtgtgtttccgtaggcaaaaaagttgcctggacaggtttacaaaacatatctccccatctccctgcagtcagcagctatcggtatctatgctaagttccttcaaagactcctaagaggtctccatggacctctgaagtttaatagtcaatgattgggtcagagcttactcagaaacctcaggccagtgaggcttccaacctctgcagcccaggctgagtggcttgagtagcacattcactgtgtggcagaactgcgagtctgcccaggcttttcatttcttctgggctccctggtgcctcccacgtgcatgtgtagaacagcattcagccagagatgcttgggaagtggatgagaacagcattcagccagagatgcttgggaagtggatgatgtctaccattctacggatcacttgcgatgcttatttcccagggaacagaaatgaagtggggccaggccatctcctgtctctgttgtctgtattacagaaggaagggagcggtgctggagcagggggcccaggagcatcacaggcggcaggccaaggagagagatgtaggtggcaggaccctccagggactcgggagagacacatgcgtgagcttttgcgatacggggtgagacagcaagggtgctgtggggtgtgtgtgccttcccccagacagtgtggatggctgcattcatgttagggctgtcataacaaagtaccgccagctgggagcgctatagaacgtcaatggattttctcacagttctggaaaccagaaattcaagatgaaggtgctgcagggttggcttccgccaaggcctctctccttggctcccagacggctgtcttctcccggcgtcctcacatgaaggtgcaaccccactatataacagtcagattggattaggacccaccctaatgtcctcattttaaccttacttaccttgtaaaggccctgtctccaaatacagccccattctggggtacggggtcggtgcagggtggggggtagggtttcaacatagagctttcaggagggcgcagttcagctagtgacagtgactgcaggtgtctaagcggagaggatgggccactccaacggggggcgggtgagcaaggggcgctggagaaagagcgtggagagcacgtgccgtctagtgtgcgcgctgggctggaaggtggggaccaggaggagaccgggaccacgagtaagagcccgcgagaggtacgtgtgagagcgactgtctccgtgtgggcgagaagcctggaaacggaggaactgggtttccgagggactgaatacctcggttgatagtctgcgcgctggcccagaaggaaggagcacaagcgcgcacgggatcccagcgtcttcccacaaccccgcctgcggctccgtccgctctccggcgccctctgctgggccagcagccgaaacgcaggggagcgctttccagcttcctccaatcccagcccacgcggtagccgctcacacgcaggtgcttaaacttaaatccatcaaaaattggcaagattaaaaaaatctcatgctggccacatttcaactgttctacgtggcatgtggctagtggcatcccttttgtacagcacagagaacatttccggcatctcagaaagttccatcagacgccctgctagtgaccaatctgcgaaaaagtgaggatcccaggctgcgcccagtggctcacgcctgtaatcccagtactttggggggccgaggcaggtggatcacctgaggtcaggagttccagaccagcctggccaacgtggtgaaaccccgtctctactaaaaatacaaaaattagctgggcgtggtggcgggcacctgtaatcccagctacttgagaggctgaagcaggagaatcgcttaaacccgggaggcagaggttgcagtgagccgaaatcacaccattgcactctagcctgggtgacgacagtgaaactccatctcaaattttaaaaaaaagtgagaatccccgactgtcccaaccacacacaacacacacacacacagcagctatctccttggttgagggcacttcccacttaggcccctccggacagtgttgtccaggacagaaacacacgtggccacacacacgccctcccctccatttatggctggcccagagctgcccagccagagagagaccacgcagggccaaaggaaataatctgctatcaaaactgaaagaggccaggtgcggtggctcacggctgtaatcccagcactttgggaggccgaggtgggcggaatcacaaggtcagattgagaccatcctggctaacacggtgaaaccccgtctctactaacaatacaaaaaattagcttagccgggcgtggtggtgggcgcctgtagtcccagctactcgggaggctgaggcaggagaatggcatgaacccgggaggtggagcttgcagtgagccgagatcgcaccactgcactccagcctgggtgacagtgcaagactccgtctcaaaaaaaaaacaacagtgaaagaaaagaaaggagtaaatgcggcttagatgaacgaataaatgcattcacccattctacctgaaatcaatacccaattgatgtaagaaacagaaatcatttaggtagatagggcgaagagagtccccagcaaaaaacttcctaacaaaaagcagcttagaaattgctccctttctcaccacaccacgcagttcaaagaaatcacttctcctaacaaagagcagcctgatctttcaggctgtaaaacacagataagcaactcgggcacagacttgggaggttcctgggtaatcaccaagccacatacatagatgggccccagtgaaaacagtgggcctaaagcacattcctttccctttctttaggcacactaagggaagctggaagcgcgtgggggagatgcctgcagctgcacgaaggtgcctgggaatgggcacagaaacactccctccccttttagcacacacagataagcagcagcgcagagcagcacaaacgaagggcctgcctgcaggatcaaagaatggggtgggggcccggcgcggtggctcacgcctgcaatcccactactttgggaggccgaggcaggcggatcacttgaggtcaggagttggagaccagcctgaccaacatggtgaaaccttgtctctactaaaaatacaaaattagccgggcatggctgcatgcacctgtaatcccgactacgcgggaggctgaggcacgagaattgcttgaacctgggaggcggaggttgcagtgagccaagatgacaccactgcactccagcctgggcgacagagcgagactccatctcaaaaaaaaaaaaaaaaaaaagaatggggtgggggctgctagagactctgctcgatgcagacagcacacctggtcctaactggttcttcaggccctaggaagaaaagacacccctcctcactagcccatctataaaacccctgacatttcttctacaacttcacaacccgttcgggacccgtctctgtgacagagctgtttcttccttttgcctattaaactcctgctccaaatctcactctgtgtgcatccacatccttgatttcctcggctgtgagaccaaaaaccttagtatttaccacagacaagaccgttttacaggaacaagccaggcagggtcccgaaagctcagtattttaagggtctaacagggagaagttctcattaatgtcagctccttctgagaactgctggggtcagaatagtccgggaaaggggagaggagacacaaggtccttgttcaaatcatgtatttcttaagatactaagagaaaaaaatacaggaaacagtatcattttttttttttttttggagacagggtctcactctgtcacccaggctggagtgcagtagtgcaatctcggctcactacaacctccgcctcctgggttcaagcgattctcctgcctcagcctcctaagtagctgggattacaggtgcccgccaccacactaggctaatttttgtatttttagtagagacggggtttcgccatgttggccaggctggtctcgaactcctgacctcgtgatccgcccgcctcggcctcccaaagtgctaggattacaagcatgagccacagcacccaggcgaaacagtatcatttctaacccttttcatgtggctgtcaggacatgtttcaagcaccgagtccagcatcttgataagatgggaaccagggagccctcagggcccccgcgccagccctcccactgcaaacccacaccaccctggccgtctggagcttgtcccagcccggctccccgtgacatcgggacctggccactcctggacgtgatgccctaagcttgcctcccctgcggatggatgtagtgatgcttgatttgggtggatgagaacattccccacaacacaagccattttgcaacctcacctcccgagcctctgagctacctttcattcccctctgagcacgcagggttaactgctgtaggggttacccccatcaatgcatgagttataccttttgacagtaacacacaacgattactagagagcatgtcattaccatttttaagtgctccaggggaggggccatgaggaggctgtaggtgaaacaggagtggttcaaatgtaaatgatggctgaacacgagtgaggcatttgcaggggtggttatgataatattgtctatagttttgtgtgcttcaagatgtccctcagaaagtttgtaattatgggccgggtgccgtggctcacgcctgtaatcccagcactttgggaggccgaggcgggtggatcacaaggtcaggagttcgaccagcctggccaatatggtgaaaccctgtctctgctaaaaacagaaaaatgagttggctgtggtcgcacgcacctgtagtcccaagtcaggagaatcgcttgaacccgggaggcggaggttgcagtgagccgagatcgcgccactgcactccagcctgggggacgagagcaagactccatctcaaaaaaaaaataaataataataataaggaaaggaagtttgtatttatggagcagtcattaaatagtgctttatgggccgggcacagtggctcaagcctgtaatcccaacactttggaaggccgaggtgggcagatcacgaggtcaggagatcgtgaccatcctggctaacacagtgaaaccccgtctctactaaaaaaatacaaaaaaattagctgggcatggtggtgggcatctgtagtcccagctacttgggaggctgaggcaggagaatggcgtgaacacaggaggcggagcttgcagtgagcagagatcgagccactgcactccagcctgggcgacagagcaagactctgtctcaaaaaaaaaaaatagtgctttaggaaattataaatatccatactaaaataatgtggatgaaacataacattatataattatccctgaaagtaaaacaaaagcatgaagaaacattcaatacaaaacaaacagcaaagggagcgatttctcggcggaaagcatgctggaaccctgtggaagcgtgggctgtcccaggacgtgcaggcaggccttagacccctgccacatacaagcaatcaccgggggtcagcacactttttgttgaagagccagatagtaaatattttaggctcaagggacactcggtctctgccacactcaatgtcaccattgccactgtagtgcagaagcagccgtggctgcactctaataaaacatttttttttacaaaagcaagcagccaatccttgggctgcagtttgagaaactccaggggcacctgtgatgtgagtaggccggtttctcaccacagtgaagggcctggcaggatggcgcttgagggatgagctggacaacccacagtcatcacagagacagacaagttctcaagaaataaaacatttctggccggacgcaatggctcacgccacacccgggaagctagaagcacgtgtgggggagatgcctgcggctgcaagaaggtgcctgggaatgggcacagaaactctccctccccttttagcacacgcagaaaaccaacgcagagcagcacaaactaagggcctgggggaggcgggagggaaggcattaggagatatacctaatgtaaatgacgagttaatgcgtgcagcacaccaacatggcacatgtatatatatgtaacaaacctgcgcgttgtgcataggtaccctagaacttaaagtataataaaaaaataaaaaatgaaatggggtgggggccgctacagtggctcacgcctgtaatcccagcactttgggaggccgaggcaggcggatcacgaggtcaggagatcgagaccatcctaacatggtgaaaccccgtctgtactaaaaatacaaaaaaaaattagctgggcgtggtggtgggcacctgtaatcccagctactcgagaggctgaggcaggagaatcgcttgaacccgggaggtggaggttgcggtgagccgagatcgtgccactgcactccagcctggcaacagagcaagactccttctaggggggaaaaaaaagggcatttcttcctattcaatgagaacatgaggaaaaggcaaaaggcagaggctggctgggagtgggtttgtgtgtgtaaaattgagtttcagtataaaaaaagatcaaggcaggactgaaagccctgaggctggcatcgcagctccagagcgaggggcaagcgtagggcgaggagcgaggatagggcgagggcgggagtagagcgaggggtaaggctagggtgagcacaggtggcaggggactctggtgggcctggactctggtgggcggggtgacccaggagctcggatgaagctcctacgggctccaggaaggttccctcaagtgccttccccacccaacccctaggccctgaacagagtcgagacccaggaatgtcccacgccccatcgcttcacctgtcccagggagaaattctggggttttttccacttcagccctctctgggggaagacgtcgggtcagaagcacatctgctcctgagagccagccgggagcaccaccatgactcttgcttagccaaacctgagggatctgaacctcctcctaggcccatccgtgcatgcccttgtaaaatcctttcagcaaatgaaccccgccgccatcccccccaacccccgccaccctcacatctgataggcttcttcagcctccaccatccccaggtgacctctgatcaccctggcctgccttcagcaagaatcctgctaggtgggtttagccgaaaacccccggacccctgaggtttgctcttagtgattttccatccactgatggtacctgtacctgtctcgatggtcctgaataaagtcttcctcacggccatttaacaagctcgccatcccactgtggggagagagacacatctgctgtagaaagagtgatacacacacagtggggggagccctcaatcggggacaacagcaggctcccagcattctcccagcgttcaaccgtgtatgtcactaagctcaggtgcttgggcctcatgggggactcctacacagcagctcctgctgagcactttggtggctggaatattctagaaagaggaataaagtaggagacacgagatctgtggtgctactttgtaattcgcactgtagggaaaagaagatgccgaagatgctgtagttaagccccaaatttatgtgcaagcctctgggtttttgtcttgtttttcaatcctgtcttctctgttttgccaaatgaggaaatggtggggagaattaaagcctcacacctttaacccctccactggactaatccaactgtatcattttatcttcgtcctcagcttttttgaagagaaagggagtgcaggctccgcagtgcgaaatcgtgaaacttatccttaatttggtgaatggagggtctgacaagtgaggggcccaggagctatgaccctgtggggagaccaagattggcaagagggaggctcggctcgcctcccctttccatgtgatcccacccagagctgccgccttcagctggctctctgtgccctgtggggctcccccatcacaaccgcctagagcagcagggtctcggacagcccaagcgtaagggacgcttgctgctgcctggggacagcaccccctcccccggtaacagtccccatttcctcctgggaaatgactctcccacaacatacccaggccgggtgtgagaagagggcttcccctccctggctaagcaagggggatgctcctctgcaactgaatctggaaccggctgaccccaaagttcctgtgtccctgggacccacctcttcctgcatggtgtggtcagcaattcctccatcaagcccccgacaaccctccagacaccctggtctgcaggggcaagtggaggccagagaacgctccgacacaggtcatgacccaattcacagcaagaaacagaaccccaacctcacatcaccccaacagcactccttttgctctgcaatccccaggtgacgtaggtctgtccaccagggagtgggcacacagggtggccacgacgctgctcggacaccgcagtcatgtccctctcagtggcctccaacactccactggctgggtgctccctggaccccgacccataacaagtgtccctgtgatgtagctgtctggccccaccctgagcccagagcgtcccccgggcagaaggggcaagaagtctgaccccaggggcctggccccacacagccttcaccccagcacctctgagacaagagctgtcggagtcactgagggagcgaacccagccgtcaggacttgaccccaggggatcacggagggagactccacatggaagaacagcctgttcggcttaaaacagacatggccagatccccatccctgaggccctggctgtggggcctgcaacaagctgtcacctagccctggagatgacagcaacacccccctcacaaggcggcccgaggattctcccggatagtctcaccaggtgtggtccagcccaggacaagagcacacagaggaaaacagcacacagaggacaaccaggaggcgcctggtggtccactcagctcagccggcagaggctgacccggctttccaggagtgcagggatggattagtgatgcttgcggtgggcccgggcgatggcgacggtgacctgtgttgcacatgtgccatctctcaggattcttctcctccctgaaccccagtgcactctctgacctcatcctggtgtcccctcaacacaagagcaaggcctcctgcaccggaagcgtctggccatgagtggcctcccgaccacctggacctgtgtgggctacagctccgccaggcctcgcacagtccaccctcaacccagccatcccttgacctgggagggtcagggaaatcagggcttctgagacagaggggctggttgccagccacccccgagaaagagatgtgacctgagccctgggtccctggatgaaggggctctgggggacacacgaaatcacagatgggaatctgggagtgccaagcccgtgggaattgccatttattcccaaagttgccaaaatcatcaccaaggattcaccgagggtgcgtgagcgggtgcgtgaggggaacgaggaggctcaaacactgactgggggttgggagtttggagggagggggaatgggtgggggccccagccacccctcccccttctaatgccacgggaaaggggtcctcctctggccagctcccctccccaggccccatgtccagtttctctccggggaggtggggtgggaaaggaagagggtgtagtgtgagtgggccccaggaaggggaagggcactgggggtggggatcccccatttcacatgcactcacaacactgatctcccagggagccggaatggggcagccggatggagccaggcccccttccgccctggattataggaggaagggattagtgttgggggccggggggcccgggggcatcatggggggcaggccagggcccccgccaaggggagagatgtacgtgggtggcgctccagggacgggaggcacaggactgagacggagctggttcagggtgagcgtcgcgggaggcgcgggctggaaggggttggtgacggaagggccagtggctgggcctccgcctggcaggaaggggttggaggccttggctccaggcggcgtggggcccggccggctcaccagcgagtccaggtcgacgagggctgcattgggccccaggaatgactccggcgtcttccgggtggggggcgtgggagttggtgtggctgcaggtggggggctgcccacagcctcagccagagatcccctgaccccactcatgtcaaacgccccagggcttcgggccggcacctctcctgccagcagctccagctctcctgcgctgctcccggaggtcggcagtgccgtgcggagtcggtcaaagtcagagaactcgtcgggctccgtgtcgaatcccccggctgttgtgccattggtgctgggcttggcaggtgaccctccccagggatctgagaaggccggggccggtgtccagggatcggaggctgagggcccactgaccgggaccccaccatcggaacttccccatggatcaggcgtgggcccctccccagctgcaggggctggggtcccaccccaagggtcaactgagggtcctgcaggggcagcaggcctccaggggtccccagaggccggcgtgggggctggacctccccagggatcagcagctggagggacaggggggccgccccaggggtccgaggtgggggcagccgtggggacggcagcagccatgggtgctgggcccccccaggggtctgtggtcggggcaggagctggggccgtgaagacgtcagcaaggtccatgagggacgactcctccttgcccccagtctccctcttgctctcctcgattgccatctgcagccgcaggtcatccccgcgacggatccgctcctcctggtcggcctcctccttgctcatggccagggccagctggagctgcagctcctcctccccgctgctctgcggccacgcctgctccgcctcgggaggggggcctgagcccacagctgctgatgaggccgtggcggtctgtgccagcttttccttggtcttgagcgcgtgcgcccgctcttcccgcagccggtcctcgtcgcgcagcagggccaccagctgcttagctttctcacgcacgttcacgccctggtccttgccgtcgcggtccacgtactggaagtccttcagcgtctgcacggcgtacatgttctccttgcactgctgcgacacgcgctccgagccggtcttgatgaggtactccatcagcgtcatggccttgtaaacgtgacgccagttcttgccatggtcattgagccgcttccagatcatgctcatgatctccgagaaggcgacaacgttgtaggtgaggtcggcaatctctgacatgagggagctggatgggccccaggggtcattgctcgtggcctctcgaaccttgatctccgcctctgagtagttgtggacgatgttcttcatctggcgcctcaaggacgaggtcgacatggtgcccggctgcagcagcaaggggcacagggccccgatgcgtggagagatggggcgactcccggacgaaggctgcggcaggtgctggcaggtcaccgcatctcggccccctcacgccgggctctggggggtcatggcggtcagccccctgccccgctcggcctcggtgtcgcgggacgtgcgccgggccacgggcgcacgcacgaacgcaaggagggccgcacgccgacggctccgccgccccgccgcccagaaggggcgcggagagccgggcgggggaggggagccgccgaggagacgggaagcaacag

SEQ ID NO: 11173 - RNA, 12226 nt, Homo sapiens
  source 1..12226: mol_type = other RNA
ctgaatagctgggactacaggtgcatgccactatgcatgactaatttttgtatttttagtagagatggtgattttgtcatgttggccaggctggtctcgaactcctgacctcaagtcatccattcgccccggcctcccaaactgctggaattacaggctcacgccacttcatgaaatgtgttgtagtggctctggattctgtatcgttctgagaggtttttttcattggtttgttttcgtttttgtgtgtttccgtaggcaaaaaagttgcctggacaggtttacaaaacatatctccccatctccctgcagtcagcagctatcggtatctatgctaagttccttcaaagactcctaagaggtctccatggacctctgaagtttaatagtcaatgattgggtcagagcttactcagaaacctcaggccagtgaggcttccaacctctgcagcccaggctgagtggcttgagtagcacattcactgtgtggcagaactgcgagtctgcccaggcttttcatttcttctgggctccctggtgcctcccacgtgcatgtgtagaacagcattcagccagagatgcttgggaagtggatgagaacagcattcagccagagatgcttgggaagtggatgatgtctaccattctacggatcacttgcgatgcttatttcccagggaacagaaatgaagtggggccaggccatctcctgtctctgttgtctgtattacagaaggaagggagcggtgctggagcagggggcccaggagcatcacaggcggcaggccaaggagagagatgtaggtggcaggaccctccagggactcgggagagacacatgcgtgagcttttgcgatacggggtgagacagcaagggtgctgtggggtgtgtgtgccttcccccagacagtgtggatggctgcattcatgttagggctgtcataacaaagtaccgccagctgggagcgctatagaacgtcaatggattttctcacagttctggaaaccagaaattcaagatgaaggtgctgcagggttggcttccgccaaggcctctctccttggctcccagacggctgtcttctcccggcgtcctcacatgaaggtgcaaccccactatataacagtcagattggattaggacccaccctaatgtcctcattttaaccttacttaccttgtaaaggccctgtctccaaatacagccccattctggggtacggggtcggtgcagggtggggggtagggtttcaacatagagctttcaggagggcgcagttcagctagtgacagtgactgcaggtgtctaagcggagaggatgggccactccaacggggggcgggtgagcaaggggcgctggagaaagagcgtggagagcacgtgccgtctagtgtgcgcgctgggctggaaggtggggaccaggaggagaccgggaccacgagtaagagcccgcgagaggtacgtgtgagagcgactgtctccgtgtgggcgagaagcctggaaacggaggaactgggtttccgagggactgaatacctcggttgatagtctgcgcgctggcccagaaggaaggagcacaagcgcgcacgggatcccagcgtcttcccacaaccccgcctgcggctccgtccgctctccggcgccctctgctgggccagcagccgaaacgcaggggagcgctttccagcttcctccaatcccagcccacgcggtagccgctcacacgcaggtgcttaaacttaaatccatcaaaaattggcaagattaaaaaaatctcatgctggccacatttcaactgttctacgtggcatgtggctagtggcatcccttttgtacagcacagagaacatttccggcatctcagaaagttccatcagacgccctgctagtgaccaatctgcgaaaaagtgaggatcccaggctgcgcccagtggctcacgcctgtaatcccagtactttggggggccgaggcaggtggatcacctgaggtcaggagttccagaccagcctggccaacgtggtgaaaccccgtctctactaaaaatacaaaaattagctgggcgtggtggcgggcacctgtaatcccagctacttgagaggctgaagcaggagaatcgcttaaacccgggaggcagaggttgcagtgagccgaaatcacaccattgcactctagcctgggtgacgacagtgaaactccatctcaaattttaaaaaaaagtgagaatccccgactgtcccaaccacacacaacacacacacacacagcagctatctccttggttgagggcacttcccacttaggcccctccggacagtgttgtccaggacagaaacacacgtggccacacacacgccctcccctccatttatggctggcccagagctgcccagccagagagagaccacgcagggccaaaggaaataatctgctatcaaaactgaaagaggccaggtgcggtggctcacggctgtaatcccagcactttgggaggccgaggtgggcggaatcacaaggtcagattgagaccatcctggctaacacggtgaaaccccgtctctactaacaatacaaaaaattagcttagccgggcgtggtggtgggcgcctgtagtcccagctactcgggaggctgaggcaggagaatggcatgaacccgggaggtggagcttgcagtgagccgagatcgcaccactgcactccagcctgggtgacagtgcaagactccgtctcaaaaaaaaaacaacagtgaaagaaaagaaaggagtaaatgcggcttagatgaacgaataaatgcattcacccattctacctgaaatcaatacccaattgatgtaagaaacagaaatcatttaggtagatagggcgaagagagtccccagcaaaaaacttcctaacaaaaagcagcttagaaattgctccctttctcaccacaccacgcagttcaaagaaatcacttctcctaacaaagagcagcctgatctttcaggctgtaaaacacagataagcaactcgggcacagacttgggaggttcctgggtaatcaccaagccacatacatagatgggccccagtgaaaacagtgggcctaaagcacattcctttccctttctttaggcacactaagggaagctggaagcgcgtgggggagatgcctgcagctgcacgaaggtgcctgggaatgggcacagaaacactccctccccttttagcacacacagataagcagcagcgcagagcagcacaaacgaagggcctgcctgcaggatcaaagaatggggtgggggcccggcgcggtggctcacgcctgcaatcccactactttgggaggccgaggcaggcggatcacttgaggtcaggagttggagaccagcctgaccaacatggtgaaaccttgtctctactaaaaatacaaaattagccgggcatggctgcatgcacctgtaatcccgactacgcgggaggctgaggcacgagaattgcttgaacctgggaggcggaggttgcagtgagccaagatgacaccactgcactccagcctgggcgacagagcgagactccatctcaaaaaaaaaaaaaaaaaaaagaatggggtgggggctgctagagactctgctcgatgcagacagcacacctggtcctaactggttcttcaggccctaggaagaaaagacacccctcctcactagcccatctataaaacccctgacatttcttctacaacttcacaacccgttcgggacccgtctctgtgacagagctgtttcttccttttgcctattaaactcctgctccaaatctcactctgtgtgcatccacatccttgatttcctcggctgtgagaccaaaaaccttagtatttaccacagacaagaccgttttacaggaacaagccaggcagggtcccgaaagctcagtattttaagggtctaacagggagaagttctcattaatgtcagctccttctgagaactgctggggtcagaatagtccgggaaaggggagaggagacacaaggtccttgttcaaatcatgtatttcttaagatactaagagaaaaaaatacaggaaacagtatcattttttttttttttttggagacagggtctcactctgtcacccaggctggagtgcagtagtgcaatctcggctcactacaacctccgcctcctgggttcaagcgattctcctgcctcagcctcctaagtagctgggattacaggtgcccgccaccacactaggctaatttttgtatttttagtagagacggggtttcgccatgttggccaggctggtctcgaactcctgacctcgtgatccgcccgcctcggcctcccaaagtgctaggattacaagcatgagccacagcacccaggcgaaacagtatcatttctaacccttttcatgtggctgtcaggacatgtttcaagcaccgagtccagcatcttgataagatgggaaccagggagccctcagggcccccgcgccagccctcccactgcaaacccacaccaccctggccgtctggagcttgtcccagcccggctccccgtgacatcgggacctggccactcctggacgtgatgccctaagcttgcctcccctgcggatggatgtagtgatgcttgatttgggtggatgagaacattccccacaacacaagccattttgcaacctcacctcccgagcctctgagctacctttcattcccctctgagcacgcagggttaactgctgtaggggttacccccatcaatgcatgagttataccttttgacagtaacacacaacgattactagagagcatgtcattaccatttttaagtgctccaggggaggggccatgaggaggctgtaggtgaaacaggagtggttcaaatgtaaatgatggctgaacacgagtgaggcatttgcaggggtggttatgataatattgtctatagttttgtgtgcttcaagatgtccctcagaaagtttgtaattatgggccgggtgccgtggctcacgcctgtaatcccagcactttgggaggccgaggcgggtggatcacaaggtcaggagttcgaccagcctggccaatatggtgaaaccctgtctctgctaaaaacagaaaaatgagttggctgtggtcgcacgcacctgtagtcccaagtcaggagaatcgcttgaacccgggaggcggaggttgcagtgagccgagatcgcgccactgcactccagcctgggggacgagagcaagactccatctcaaaaaaaaaataaataataataataaggaaaggaagtttgtatttatggagcagtcattaaatagtgctttatgggccgggcacagtggctcaagcctgtaatcccaacactttggaaggccgaggtgggcagatcacgaggtcaggagatcgtgaccatcctggctaacacagtgaaaccccgtctctactaaaaaaatacaaaaaaattagctgggcatggtggtgggcatctgtagtcccagctacttgggaggctgaggcaggagaatggcgtgaacacaggaggcggagcttgcagtgagcagagatcgagccactgcactccagcctgggcgacagagcaagactctgtctcaaaaaaaaaaaatagtgctttaggaaattataaatatccatactaaaataatgtggatgaaacataacattatataattatccctgaaagtaaaacaaaagcatgaagaaacattcaatacaaaacaaacagcaaagggagcgatttctcggcggaaagcatgctggaaccctgtggaagcgtgggctgtcccaggacgtgcaggcaggccttagacccctgccacatacaagcaatcaccgggggtcagcacactttttgttgaagagccagatagtaaatattttaggctcaagggacactcggtctctgccacactcaatgtcaccattgccactgtagtgcagaagcagccgtggctgcactctaataaaacatttttttttacaaaagcaagcagccaatccttgggctgcagtttgagaaactccaggggcacctgtgatgtgagtaggccggtttctcaccacagtgaagggcctggcaggatggcgcttgagggatgagctggacaacccacagtcatcacagagacagacaagttctcaagaaataaaacatttctggccggacgcaatggctcacgccacacccgggaagctagaagcacgtgtgggggagatgcctgcggctgcaagaaggtgcctgggaatgggcacagaaactctccctccccttttagcacacgcagaaaaccaacgcagagcagcacaaactaagggcctgggggaggcgggagggaaggcattaggagatatacctaatgtaaatgacgagttaatgcgtgcagcacaccaacatggcacatgtatatatatgtaacaaacctgcgcgttgtgcataggtaccctagaacttaaagtataataaaaaaataaaaaatgaaatggggtgggggccgctacagtggctcacgcctgtaatcccagcactttgggaggccgaggcaggcggatcacgaggtcaggagatcgagaccatcctaacatggtgaaaccccgtctgtactaaaaatacaaaaaaaaattagctgggcgtggtggtgggcacctgtaatcccagctactcgagaggctgaggcaggagaatcgcttgaacccgggaggtggaggttgcggtgagccgagatcgtgccactgcactccagcctggcaacagagcaagactccttctaggggggaaaaaaaagggcatttcttcctattcaatgagaacatgaggaaaaggcaaaaggcagaggctggctgggagtgggtttgtgtgtgtaaaattgagtttcagtataaaaaaagatcaaggcaggactgaaagccctgaggctggcatcgcagctccagagcgaggggcaagcgtagggcgaggagcgaggatagggcgagggcgggagtagagcgaggggtaaggctagggtgagcacaggtggcaggggactctggtgggcctggactctggtgggcggggtgacccaggagctcggatgaagctcctacgggctccaggaaggttccctcaagtgccttccccacccaacccctaggccctgaacagagtcgagacccaggaatgtcccacgccccatcgcttcacctgtcccagggagaaattctggggttttttccacttcagccctctctgggggaagacgtcgggtcagaagcacatctgctcctgagagccagccgggagcaccaccatgactcttgcttagccaaacctgagggatctgaacctcctcctaggcccatccgtgcatgcccttgtaaaatcctttcagcaaatgaaccccgccgccatcccccccaacccccgccaccctcacatctgataggcttcttcagcctccaccatccccaggtgacctctgatcaccctggcctgccttcagcaagaatcctgctaggtgggtttagccgaaaacccccggacccctgaggtttgctcttagtgattttccatccactgatggtacctgtacctgtctcgatggtcctgaataaagtcttcctcacggccatttaacaagctcgccatcccactgtggggagagagacacatctgctgtagaaagagtgatacacacacagtggggggagccctcaatcggggacaacagcaggctcccagcattctcccagcgttcaaccgtgtatgtcactaagctcaggtgcttgggcctcatgggggactcctacacagcagctcctgctgagcactttggtggctggaatattctagaaagaggaataaagtaggagacacgagatctgtggtgctactttgtaattcgcactgtagggaaaagaagatgccgaagatgctgtagttaagccccaaatttatgtgcaagcctctgggtttttgtcttgtttttcaatcctgtcttctctgttttgccaaatgaggaaatggtggggagaattaaagcctcacacctttaacccctccactggactaatccaactgtatcattttatcttcgtcctcagcttttttgaagagaaagggagtgcaggctccgcagtgcgaaatcgtgaaacttatccttaatttggtgaatggagggtctgacaagtgaggggcccaggagctatgaccctgtggggagaccaagattggcaagagggaggctcggctcgcctcccctttccatgtgatcccacccagagctgccgccttcagctggctctctgtgccctgtggggctcccccatcacaaccgcctagagcagcagggtctcggacagcccaagcgtaagggacgcttgctgctgcctggggacagcaccccctcccccggtaacagtccccatttcctcctgggaaatgactctcccacaacatacccaggccgggtgtgagaagagggcttcccctccctggctaagcaagggggatgctcctctgcaactgaatctggaaccggctgaccccaaagttcctgtgtccctgggacccacctcttcctgcatggtgtggtcagcaattcctccatcaagcccccgacaaccctccagacaccctggtctgcaggggcaagtggaggccagagaacgctccgacacaggtcatgacccaattcacagcaagaaacagaaccccaacctcacatcaccccaacagcactccttttgctctgcaatccccaggtgacgtaggtctgtccaccagggagtgggcacacagggtggccacgacgctgctcggacaccgcagtcatgtccctctcagtggcctccaacactccactggctgggtgctccctggaccccgacccataacaagtgtccctgtgatgtagctgtctggccccaccctgagcccagagcgtcccccgggcagaaggggcaagaagtctgaccccaggggcctggccccacacagccttcaccccagcacctctgagacaagagctgtcggagtcactgagggagcgaacccagccgtcaggacttgaccccaggggatcacggagggagactccacatggaagaacagcctgttcggcttaaaacagacatggccagatccccatccctgaggccctggctgtggggcctgcaacaagctgtcacctagccctggagatgacagcaacacccccctcacaaggcggcccgaggattctcccggatagtctcaccaggtgtggtccagcccaggacaagagcacacagaggaaaacagcacacagaggacaaccaggaggcgcctggtggtccactcagctcagccggcagaggctgacccggctttccaggagtgcagggatggattagtgatgcttgcggtgggcccgggcgatggcgacggtgacctgtgttgcacatgtgccatctctcaggattcttctcctccctgaaccccagtgcactctctgacctcatcctggtgtcccctcaacacaagagcaaggcctcctgcaccggaagcgtctggccatgagtggcctcccgaccacctggacctgtgtgggctacagctccgccaggcctcgcacagtccaccctcaacccagccatcccttgacctgggagggtcagggaaatcagggcttctgagacagaggggctggttgccagccacccccgagaaagagatgtgacctgagccctgggtccctggatgaaggggctctgggggacacacgaaatcacagatgggaatctgggagtgccaagcccgtgggaattgccatttattcccaaagttgccaaaatcatcaccaaggattcaccgagggtgcgtgagcgggtgcgtgaggggaacgaggaggctcaaacactgactgggggttgggagtttggagggagggggaatgggtgggggccccagccacccctcccccttctaatgccacgggaaaggggtcctcctctggccagctcccctccccaggccccatgtccagtttctctccggggaggtggggtgggaaaggaagagggtgtagtgtgagtgggccccaggaaggggaagggcactgggggtggggatcccccatttcacatgcactcacaacactgatctcccagggagccggaatggggcagccggatggagccaggcccccttccgccctggattataggaggaagggattagtgttgggggccggggggcccgggggcatcatggggggcaggccagggcccccgccaaggggagagatgtacgtgggtggcgctccagggacgggaggcacaggactgagacggagctggttcagggtgagcgtcgcgggaggcgcgggctggaaggggttggtgacggaagggccagtggctgggcctccgcctggcaggaaggggttggaggccttggctccaggcggcgtggggcccggccggctcaccagcgagtccaggtcgacgagggctgcattgggccccaggaatgactccggcgtcttccgggtggggggcgtgggagttggtgtggctgcaggtggggggctgcccacagcctcagccagagatcccctgaccccactcatgtcaaacgccccagggcttcgggccggcacctctcctgccagcagctccagctctcctgcgctgctcccggaggtcggcagtgccgtgcggagtcggtcaaagtcagagaactcgtcgggctccgtgtcgaatcccccggctgttgtgccattggtgctgggcttggcaggtgaccctccccagggatctgagaaggccggggccggtgtccagggatcggaggctgagggcccactgaccgggaccccaccatcggaacttccccatggatcaggcgtgggcccctccccagctgcaggggctggggtcccaccccaagggtcaactgagggtcctgcaggggcagcaggcctccaggggtccccagaggccggcgtgggggctggacctccccagggatcagcagctggagggacaggggggccgccccaggggtccgaggtgggggcagccgtggggacggcagcagccatgggtgctgggcccccccaggggtctgtggtcggggcaggagctggggccgtgaagacgtcagcaaggtccatgagggacgactcctccttgcccccagtctccctcttgctctcctcgattgccatctgcagccgcaggtcatccccgcgacggatccgctcctccttatcatgctcttctcggctcaaactaagggccagctggagctgggcgtcgtcctcggggccgcaggacgggggctggtcggcctcctccttgctcatggccagggccagctggagctgcagctcctcctccccgctgctctgcggccacgcctgctccgcctcgggaggggggcctgagcccacagctgctgatgaggccgtggcggtctgtgccagcttttccttggtcttgagcgcgtgcgcccgctcttcccgcagccggtcctcgtcgcgcagcagggccaccagctgcttagctttctcacgcacgttcacgccctggtccttgccgtcgcggtccacgtactggaagtccttcagcgtctgcacggcgtacatgttctccttgcactgctgcgacacgcgctccgagccggtcttgatgaggtactccatcagcgtcatggccttgtaaacgtgacgccagttcttgccatggtcattgagccgcttccagatcatgctcatgatctccgagaaggcgacaacgttgtaggtgaggtcggcaatctctgacatgagggagctggatgggccccaggggtcattgctcgtggcctctcgaaccttgatctccgcctctgagtagttgtggacgatgttcttcatctggcgcctcaaggacgaggtcgacatggtgcccggctgcagcagcaaggggcacagggccccgatgcgtggagagatggggcgactcccggacgaaggctgcggcaggtgctggcaggtcaccgcatctcggccccctcacgccgggctctggggggtcatggcggtcagccccctgccccgctcggcctcggtgtcgcgggacgtgcgccgggccacgggcgcacgcacgaacgcaaggagggccgcacgccgacggctccgccgccccgccgcccagaaggggcgcggagagccgggcgggggaggggagccgccgaggagacgggaagcaacag

SEQ ID NO: 11174 - RNA, 2191 nt, Homo sapiens
  source 1..2191: mol_type = other RNA
ctgaatagctgggactacaggtgcatgccactgcacttggttcaagggagaccttttaaatcatcatagaaataaagatgttgggcaaactgatcaactatttggaaaaaaatttacatctgacaccatatattgaatatatgttgccaaatgtaaaataacaaaatcaaaacttatgtgagttgatttgtcttatcttaggaagagcaaagaattttaagcatgaatgcaatggcagaaaccaaaaagctttctagatttaaaatcgaattttctttaaaataaataaaaaaccataagaagtccaaatagcataagatgtgtgcaccttggaaaaaggttttttttcttacataaaacaaaattttaaagtaaaaaaatttttttaaagtttttttgcacttattcagtgcacgtgatatgccagaaacaatgccaggaaccaggaattcaaagataaataagaaacaatcactacatttgagcatctcatatctagtaataaaaatagtaatttatataattgttagaacaatgctagagtagaagattgacaaggggctgtgacaacccagggtagagaagtctcagacaacatgattcttaggaagggacatgagatattccacaggaccaccaatcctcttttcggcaagtggtcaaaagtgggctaccattttttcctgtgttccactctccagtagcatgaactgagaccagggattccaaacataaccctgtgaagaccccctctggctcgcttactctctctagatcaccccactttataccctagagattaccttgtctgtggtggcactattttggtggcacggctttgatattaaggaagatgatggtcagaaaaagaaagcagaaaatatcttctaattttgaaccctactttatgtcaggcactatgctagcacaatacacactagaactctctaaggtagatattgtattattatttctacttaaaataaagaggctgaggtccagaaagtaaatctgagttctgtgcctatttaatctagatgacctctgcttacctgcttgcagggagtgcacatcaaaggaagactcaaggtggcaggaagcttgctgtttatttcaaacttaaaatagtggctgaaagagggtggtgattttgacctccttgtggagcatgaggagctcaggagagcatctccttcccgggctttcagaaagttgtttcatttcttaggtggtaacctattatatagaccttccttggtaaagtctttccacctttcagctattctccatcagctgctcaccatgattcttgggagaaggcaaaacctgttttctctcagcagagaatttcccatcctctcagtcctctcagggcttcccctccgtccctttaccacttccttcttgccttgtgctctgacagggcaactcctgacttaaagaaagggctgtgtggctctggccacccgtgcagagacagcagaaaggagaagggtgtctctgcagagggaaggaagaggctgggggaggagtgttagaggcacgcatgtgcagaatgtcctaacatgtcagtgcctgaaccaacctggctgttggccataaccagcaactacccgtcaatgagagcttcgaacctctggggaatcccaggtctgaaattacagatgggccatgggagtttttccactacagatatttacgtttataaatcacgttgtcttcttagaaaagtcagaaggaggttaaaacagtcaagccacagacctgtagaaaatatagtatcaacaactctcaaatctgaaaacaaacacccagtaacaaaatgggcaaaatatttgaacagacatttcaccaaaggaactatacagatgaacattaaaagatgctaaacattgtagttattagggaagtgtaaatcaaatccacaatggaacacttttacatacttattacaatggctataaaaccctgacaatatcaagtatggcaaggtatgcaaagcaactggaagtctcatgcattgctgatgagaatgcaaaatgacagcctttttggaaagaagtgataaggacagaaggcagggctttactgggtagaagagggtggttcactggcaaaggtcccaccctcaagccttgaaaccgaagccctaaatgagaacagttatccctgttatcctgcccaaatgtta

SEQ ID NO: 11175 - RNA, 3783 nt, Homo sapiens
  source 1..3783: mol_type = other RNA
ctgaatagctgggactacaggtgcatgccagcgtgaccagctaatttttgtattttttgtagagattggggtttcaccatgttgctcagacttgtcttgaactcttgtactcaagtaatttgcctgccttggcctcccaaagtgctggaattacaggcatcttgtttttttatttttaagtagagatagggtcttgctatgctgtccaggctggtcttgaactcctggcctcaagtgatccaccagcctcagcctctcaaagtgctgggattacaggcgtgagccaccatgtttggacaacttttatttatttttttgagacagggtctcactctgttgtccagggtggagtgcagtggcatgatgagagctcactgcagcctcaacctccaaggtccaagcaattctcccacctcatcttcttgagtagctgggaccacaggtgtatgctaccatgcttagctaatttttaaatttttttgtgtagacagagtctcactatgttgccaaggctggtcttaaacttctgggctcaagcaatcctccccgcttggcctcccaaagtgctgagatttcgggcatgagccaccacacccagccaagattgcgttttttatttggttctcagcttgaatgttattggtgtatagaaatgctactgacttttctatgttgattttatatcctcaaactttactcaagtagtttatcaggcctaggagttttttggaggaacctttaaagttttttaggtacaggattatattttcagtaaacggagataatttgacttcttcttttcctatttggatgcctttcatttctctctcttgcctgattgctctggctagggctttcagtactatgttgaataggagtgctgagaggggacatccttgtcttgttccagttctcaggaagaatgcatacaacttttgctagtttattatgatattggctgtgggtctgtcacagatggctgttattattttgggctattttccttcaatgcgtggtttgttgagtgtttttgtcataaagggatgttggatttattgactattttttctgtgtctattgagatgatcatatggtttttgtttttagttctgtttatgtggtgaatcacatttattgattcgtgtatgttaaaccatccttgcatccaggtttaaagcccacttgatcgtggtgaattatctttttgatgtgctgctggattcaacaaccaattttcttaatgatacatgggagttgagggactcattaactataggaagtgggcttgaacacattttttacagttctcaaatacctctaaaagtcattttcttggatataggtgaggggagtgaaacctgtgaaggagacaatggaaagataaataaaatattataggtttactagaaaaggaaaaaccaagacattaataaaccacgtcatcattcgccgaataccttataaaagggcagtatcacaccattgtagactcttactttgtcattttcttcatcatatcagtagtaaggcaattttgtatcaatataaggaatctgaacacaaatatgaattgccttcatagatcatggtttttcttttaaaatattggcagaaacagaaaagttctctgttaaataatctatttttaaggaaatattatcaaaggaaaatataagataaataatatcaactctttgattacgctttgctctttttttctaggaaagctaagacaaaaagtaatacagccttaattcaaacaacagagataatatctctgcacatttgtcttacacttttatttaatgtttacacacattttaactacattttattgacaaatacaaggagacattttaatgatgcttttagttttataacatgtttttcctggtgacattgaagaaaaaattttagatatattaattaagatacatagtttaaacatttcatataaaattaatttcatagttgaatgtggttttagtaagtttttaatttatagctacctctattttatgaatgaagaatctattttgcctttattttattattattttttattatactttaagttttaaggtacatgtgcacattgtgcaggttagttacatatgtatacatgtgccatgctggtgcgctgcacccactaactcgtcatctagccttaggtatatctcccaatgctatccctcaataaaccatagtaattattaatttacctaaaatttagttacataggtgagagagcgaacactttctatatagtttagaagagctaaatcttggtttttaggctaatttcattaagaagtgttgatgatatgtaactatgtctaactaaaagtgtgaaataaggtgtttagaaagagttcatgtagagaagggtagagagtttttcattcagctttgcctttgggggtacattttttacataatcacattcatttatttaaagaaaaaatcatcttctggaccatgctcttgaaggcttgcttcacttgcttatttctcagtgtgtatatgaagggattcaagagaggagccactgaggtattgagcacagctactcctttgcttaaagtcaccctttctctggcagaagtcttaatgtacatgaagatacagctactgtaagagatggagacaactatcatatgggaggagcaagtggaaaaggcttttttcctttgactcatagaaggaattttcagaattgtccggatgatgtttgtgtaggagagaataactaatgtcaaggtgaccatcagtgttaccacagctaaaaaaaatgccatgagttctagaaagtgagtgtttgtgcaagagagctgcagcattggagaagagtcacagataaaatgatcaattacattggaggcacagaaatccaactgcagcagaagcattactggtggaaagatgatcagaaaccctgcaagccaggagctaaagacaagaagggtacacactctggtgctcatgatgattgtgtaatgaagaggtttgcagatggccatgcagcggtcataggacatggcagccagaaggtaaaattctgtcacccccaagaagatgaaaaaaaatagctgagccacacacccattataagaaatggttctgtttcctgtcacaacagtgacaaggaatctgggaatgcagacagacgtgaatgaaatttccaggaatgagaagttccgaaggaagaaatacatgggagtctgcagatggggatctgaaagggtgagggtgataatgatcaggttcccagtcacacttaacatgtaggtaacaagaagaaatatgaaaagtacaacctgccactgtgggtcacttgtcaatccaagaagaataaagtctgttactgctgtggaatttctcattatttttttctttagaaaagtattctgtattttcgctgtaaaataggtgaagaaaccagaaaactatgacaccagtaaagaaaattattattttttttctgtctggctctttccatttaccataatgccttccaggttcatccgtaatgtcacaaatggcagtgtggcagtatctccttcttttatgaggctggataacattccattgtgtctagctatccgctgatgcatctatcttataaatcaattatttctgtatttccttcattatatttttatatatttcagaatacatctctgtcttctaaatgtttcagtatattccctatcgccgctttaaaaagtattaccttgatacaaattttagttgaaatgaaggctaatgtagtggctttccgag

SEQ ID NO: 11176 - RNA, 1596 nt, Homo sapiens
  source 1..1596: mol_type = other RNA
ctgaatagctgggactacaggtgcatgccagtacgcccagctaatttttttgtatttttagtagacatggggtttcaccatgttggccaggatggtctccatctcttgacctcgtgacccgcccgcctcggcctcccaaagtgctggggttacaggcgtgagccactgcgcctggccacatcatctcatttttcaagagatgtgtcttttagaaaatttgcattttttaaaattatactttggtctgcaaaaaattgcatttttaaatgtttgccactaattgattcttctcccctcaaaatggcagtgcaagtcaaaataagacacaggcagccagttcgcaacctgttgtatacactccacaataaaaataaatggatccacacagtagcaaaatatgtgtacaaaacctaccaggaagaccagggacagacccctaccctccggtcaacatgagacaaggagagggaaggaaggctgagaatggggcaggagcccttgcagcaccagcctgtgtctgcagccctgggtcctgaggtaccactgggggatggaagaactccaaggagagccccagctgggtcctaataccccaggagccttctggcttcttcactttgggcctgcagggtctcgcttgcatacttctggaggagttccattttcttccttcgcaccagtgcctcctcaatctcttgctgcgagggaacagggacgtgagcaatgaacttctgctggctgtcgtcccctcctttctcctggctgccttcctcgtccgactcctcctcggtgactgcatagatgttgatctcttcctcctcttcctcctcctcttccttttctcctcttgccagccgagcctctctctctgctttccacttttccactaactcggctctgagtttcttttcatattcctgttccaaaggcacaataacaccatcatcttcatctaggtaaccatagtactcaaaatcgattgccttcatgagctcagcacgtgtctttctgggaggaggaagagcttgtgatccgcccgcctcagcctcccaaagtgctgggattacaggcatgagccaccgcacctggcgttctttttcaaacagctctctaacaccaggcaaatcttttgctgctccaaagtacttgtaacctcggtttcctgggacttcttttccttcatgatccagcattttagggccaacttttccataatcaggacctcccagctcctttatccggacctcccagtgtcctttctcccttagcagcttgttaatttcatcattcaggtcacgaattcgaaattcacctaaaccagcattctgaatctgagccacttttttagagatctctccaatgatctgtcgtctccacttctcagctttaggcagttcagtacattctgaggccagaaagggtcttcgttccttcacttttccctcttccagctgagcctggcgaaatcttgctaaggccgtcatggccttttctgcatttcgggccatggtgtcgctaagggcgccgtcctggagccccgcggcccctgtccaagaaactccacaggcccagaagacgccgacgctcacaggaact

SEQ ID NO: 11177 - RNA, 1530 nt, Homo sapiens
  source 1..1530: mol_type = other RNA
ctgaatagctgggactacaggtgcatgccagtacgcccagctaatttttttgtatttttagtagacatggggtttcaccatgttggccaggatggtctccatctcttgacctcgtgacccgcccgcctcggcctcccaaagtgctggggttacaggcgtgagccactgcgcctggccacatcatctcatttttcaagagatgtgtcttttagaaaatttgcattttttaaaattatactttggtctgcaaaaaattgcatttttaaatgtttgccactaattgattcttctcccctcaaaatggcagtgcaagtcaaaataagacacaggcagccagttcgcaacctgttgtatacactccacaataaaaataaatggatccacacagtagcaaaatatgtgtacaaaacctaccaggaagaccagggacagacccctaccctccggtcaacatgagacaaggagagggaaggaaggctgagaatggggcaggagcccttgcagcaccagcctgtgtctgcagccctgggtcctgaggtaccactgggggatggaagaactccaaggagagccccagctgggtcctaataccccaggagccttctggcttcttcactttgggcctgcagggtctcgcttgcatacttctggaggagttccattttcttccttcgcaccagtgcctcctcaatctcttgctgcgagggaacagggacgtgagcaatgaacttctgctggctgtcgtcccctcctttctcctggctgccttcctcgtccgactcctcctcggtgactgcatagatgttgatctcttcctcctcttcctcctcctcttccttttctcctcttgccagccgagcctctctctctgctttccacttttccactaactcggctctgagtttcttttcatattcctgttccaaaggcacaataacaccatcatcttcatctaggtaaccatagtactcaaaatcgattgccttcatgagctcagcacgtgtctttctgggaggaggaagaggttctttttcaaacagctctctaacaccaggcaaatcttttgctgctccaaagtacttgtaacctcggtttcctgggacttcttttccttcatgatccagcattttagggccaacttttccataatcaggacctcccagctcctttatccggacctcccagtgtcctttctcccttagcagcttgttaatttcatcattcaggtcacgaattcgaaattcacctaaaccagcattctgaatctgagccacttttttagagatctctccaatgatctgtcgtctccacttctcagctttaggcagttcagtacattctgaggccagaaagggtcttcgttccttcacttttccctcttccagctgagcctggcgaaatcttgctaaggccgtcatggccttttctgcatttcgggccatggtgtcgctaagggcgccgtcctggagccccgcggcccctgtccaagaaactccacaggcccagaagacgccgacgctcacaggaact

SEQ ID NO: 11178 - RNA, 7969 nt, Homo sapiens
  source 1..7969: mol_type = other RNA
ctgaatagctgggactacaggtgcatgccatcttgcccagctcatttatttttttgtatagacggcataaccctgtgttaccccgttggtattacaggcatgagccactgcacctagccaggcatattggttttaaaagggttacaagaaacaagatgcacttttaggcctcctataatcctgcatttccaaagcatccatttagtcatctcatcaaaattttcattgatttaaataagttaatatgaacagactgacataattttactttaatgatgttgtttattgtcctaagccatccatacacaaaacgtttaatgtgttatggaaggctaacagtttttcagcttttctcaatactttcagccatccatacataaaatgtttaatgtgttatggaaggctaacagtttttcaacttttctcaatactatcagatgaatgtattcttaccaatcatgatttacgtttttcaaatgtggatttcttaggcctttgactgatagctttaggcttttgcactacacaaagaaaaagacacctttctattcatttcttaataatttgtttccataaagctaaaatgtccactgatgacataatctacctttggttaatcacagcaaatagttcacattttaaaggaatgcagatatttggatagaagcctctaacaatgtaaatattgtgcatttcaagttccatagtgtgtctaaccagggatagcaactgattatatgtggattaacaatagtgaataactgagcacatattaacatgaataacatacacagcagtcaaaacttactgtttttcatatgtgtaaagtaaaaattcaatctatctttaaccggctcatactgttttcatgttgttcaactatttgacacaaaaggagctttttcctttctttaaaaggattttgattcagtcataacagatttttgaaagtgacagtaaaattatgcatttggtccaggattaagagggaagttttgcttgctagtgtctatctggttagacatcagaataaaatgaatggactgtaaaggatcttataaccagtctctctctttaatatgaaggcccaacattacataattctttttaagagttgaccaggaatgaaatgtaacctcttttaaagatgaagaaaaactgaaaaaatgagattaagaaaatatgtgggtagtttacagctgctgatagaattgtgtgcacgcgtgcatgcatgcataaacacaaagtgaatctagaagggaaaaaattgagtttgatgaagtctaagatgaaaggttccatttcatgtaagattatgtgaccttggaaaaatttactggcttgctagtggaatacgtccttatatagggacttgaagagtttatctaaatagactgacttaaggatgcttttcctcttgttagacttgtatgacattactgagaagatttagagttctagaagtagagaagactgattagcttgtgcctgtgtatgaagaatgacaaattaagacaaaaggttatgtaaaccatttactaaaaaagtctaaatttttatattcctaggcccctacttatcttttacaaactttgaaggacctgaaattctttggacaccatcagatttagtttataagagttctgattttgaatcaagaaattattcatgtagttttaaaacacaattaaaattttcagtcaggctgaacttttgtgcacttcctcatttattcgagaaaccccaccactaatgtatttagaccttaatatgatggctttgagtcttaaatcattgtccacctaaaataatataccaaataaagatttttaaagtgctgcatatggtttctgtaagaggtacataattagattaccagcattatcctttagcttcaaaagtaaaactcatagtcaggattttactgatagtacaggaagaaaaaaaataaccactgttgaaaaataaatgaaaaaaattttattgagtattactttatacatgcaaattgaaagtgaatctatattaagttgactattccacaataaaaacctatgaaatgggaatgatcaaagctgtctaacacaatactaatgtgttcaataaattatccagatgtttttccacaaatatttggattacctgaattagctgattcttcagcaaaagttaaattttagctttaatatggtagcagcaggatgctacttaaatttagaagaaaaacataagaataaaaaccctgaatagcatagccaaatcttccaagaaataagttcaccaaaaaagtagcatacacctatttggtatccagaggaggaaacaaaacacaggcacttaatcaacatccaccaagtgatcatcactaacattctattattaccagagtaactgtcgatatgtgaactgtagattagaacagacttacatatctaaaaacaaaccagtaatcaataatatatacagaaatactaacttgaagtcacatttaaataccatcaacagtttggtgtatctgatataactgaattcatttcatcactgctataaattccttaaaagtgttcttttcctaattaacattatctttaaaaaatggtagatatttcccagtatgcatcagttttttcactccaccattcagtaaatgttgtagcaaattaaatagaacctattaactagatctaaaaacagtggctgaatacttaacacaaagaagtacttttgagtaaactattcagattagacaggctaatgctaagactgcattttgtgctactgacatgcactatatagatcgtacactactagatggaaagttggtccatgtccatttatttaaagattctgtaacacctgtaatagtatttaatacagctcccacatactatattcctctcacatagacatagttatttttagtggggataaggatatgactttaacatgctatgagattctagctaagtaaaataaaaacaatatggactcagattttcttaggagatattagttcaagtttttaaactgggaaacaatcaacttccatatatccaggagaaacttagcatggggggaggtgccttagttgatgtgcctgataagcaaactgttagttgtctattagtattatgttttcggcttaatgtaacaacaaaagaaagttgtcacactacctctcagataatatcaattacaatcttagagactgtaattgggaatacaatcctataacaagttattaacaatatcatgaatagttattaagtaagtgccagcactacatgcaacttactggtcaccaactcagaacccataaaactatacacatatgcacaaaaaaaaaactccaaagaaagatacctatcactgtacatatgaatactgtccaggatatcagatcaattatcaaatccaaggtctctgctgttttgtcttacagtgttgaatatatgaatgcttctctattacactgacttgtactattttcaagaaattaagtggattcaaaatcttacatttttatttctaattataaaatccagattaatccaaaaaacacaaaccacatgtaaccgaggtaggtttttcaccttaagaatacattgcttctaccacaattaaaaattttttaaactgaagaaaaaaaaaaactacattgctccacatacctgatacttaattttctatgtttgaaactacttgaacaagtgtgacagtgctaatctactatatttagtaaatcccttagtacctataaatacacacccaaaagcccttccctccttctctaatggtaactgttgtataataaaattgtcaacaactctagaaagatgaaataaagattactatagcaatcttcaattaattcatttcagaaatcaaggaggcaagtcatgttcattttaaagatgacaaacttactattttgaaaatgagctcataaatacattagaactttgaatgtgctttattatgccacaaattcccaggagatttaagaaatagtatttctgaacaggaataataatttcacaaatactaacactttattgacaatagacaagtcttttagggtagtgcacatgtacttaaaaactaccttctaccaatctcaacactttttataaattttcaggtgaaactgtagcagatcctactttatttttcaatggttagtgtaaaattctgtatgtaaaataagtacatattttgagatggaagaaggactgcatgtgaaatgctttgcctaagttgtaaggctcctgtctttacgctatcattaaaggccaaaaaaatcactgctagaaatgttccccaaaaaattcttaaacagctcagtctttaaaagtattaataatttttttttttttttttttggagacagagtttcgctcttcttgcccaggctggagtacaatggcgcaatctcagctcaccgcaacctctgtctcctgggttttcaagcgattctcctgcctcagcctcctgagtagccaggattacaggcatgcgccaccacacctggctaattttgtatttttagtagagacggggtttctccatgttggtcaagctggtctcaaactcccgaactctggtaatccacccgccttggcctcccaaagtgctgggattacaggcatgagccactgcacccagcctaataactgatataatttttttaagtgaaatgaaatgttcctttatttacatatgaattaaatagaaaattcaaagtaattcttttaataaaaacccatatactaatatattttaaggttggatactaacagcattttcacaagatccaaagtgtggatgacgaactaggcaataaggacatgtgtgccacataactaagggtaactaaaggaagatgagtacctcacaaccaaaagcagttaactatgcctggcataccaccctgtcatgtgggcagatcactgttcccatgctgggtaagagtctccaagaagggaagcccttatgcagtaattctgtaactatattaaatttggtaatctaacattaaactttttcgtgagcagtgaatatacacatggtcatatgaaaactgccctggagaccgggttaattattaaataaactaaaaggggagaaatgctgatagataaaattatgtcaattccagggtgttcaatggaataaagaaacagcagcagctgcttcaaaagtagactatgatcagaaacctcagatggtaacctttaaaaattgtggaatccagagtctcaacctaaacctacataggagctacagccagggagttctttctaagttcctcaagtgattctgatgattggccaagctggaaacttctgaactgggggagaaagccaacctaggtaaatgtagagacttttagaattcaacatttgattatcatttactccacattttcccccagctgtctcaccttctctatttttctaacagtgaacaataaaagggcttggcaagtgaaggaaaaagtcagtagagtacctaaaatggatttgactatattcaagccactttcatatattaactagataaaaggataccatactgctatttgaaattcaatcacaaagcaaaaatgtcataattttaatgtattttaagggaagacggggttcttaacatgaatatgtaatacaaaaacaattctaaataataatatttaatagaagaaaaaatctgtataattatttagaagtaactctgtttttaaaatttcaatgttaggaagaaaatcccttaaatttgaaatagcggaatattctctcatatgaaaaaactgtgtcccagtgttattcttcaacttagaaattaggcaaagtattttagtactatttctgcttacatattgttttgtatgaatgttttaagtatgaataatattttggtttttagtgtgcatgctaatataaaaatatggatttttttctcctacactgactttgtacactttccaggcccgaagaataaaaaacttttaaaatatcctgtgttcactagcaaaccttggaacgataaaaaaaggtagtacctacataagaaattttacattgaaattacaattgtatgtttttcaggagttaaagtgattcaatttttcaatattcaaacacaaaatagtaaatttttatttactatagcacaattcaagtattctcttaaatttatatttagtcaactaaaacatgacagtgactttataagagctttccttttaaaaggttgctgttataaaaaagtatgactctattactctaaatgcttagaataagtggaaagaacaaatgacagtagacaaaaacctttatgagtgagtcatcaacacataaaaggttgcacacatcagtaataggacatgtgaaggtaacatcccaaaagtatttgaactcatgtaaacaaagactatgtatattcctaagggagaaaatgtactaccaagataaaatatattcaaacggctgtgactttaaaccatgtattagttgaataccacacaaaaccaaaaaggcattatctatcatttaataactgaaagatattacttatttgtgagataaaaggataatgcttttttaaaaccaataatgaaaaagaagtattttgaaaacaaacatctgtttgctagaaataaatatacttgcttagttattttaatgtattgcagcataggaatattgtgctagcattgaccattaacattcaatcagtagtttaaaatattttttccacattgagtcttgaatcctctacctggtcagctgacccacaactttcaaaagagttttattttcctgctttagctgttcattttcatcttctatgtcatctaggtctctatttaataaatcaatttcttctttgagttttccaatcatttcctctttatcttgcatcagtctcacaagtcttaggttttcttgtctttctcttactacttccttttcaagatcttcaattttcttttccagtgtgctacttgaaaccagagtacctgaaacatttgcatccctgttatatctagggaacccacttctatctgttcgagaatatctacttgagacatcttcttcagagacactggttgtgcttttatatctgcctgaaactgttctaggtggctcctgtagcagataggaactgcctggatctagtaagtttacagcttcattctgaatagtgttctgttgtgtaattgcatcttctcgtttccgctctttctgccctgcttcatcatcttcgtactcatctaagcactctgcggcagggatgttgaccacgccggtggagcgccgcttctcccgcagcttcctcttctcgatctgccccttgcctttcctggcactggggcccgagctcttgcccttctctgggacgccgtccggctcctcctcgtcacgctggggcggcggtgcagccgaggcagaggcggctgggggctcgtcctccgaccgccgcgggccgggggccgcccgcgtcagcatggcggagccgaccgcgcagttcacgcccccgggaccggggacggcaggtgcggccggcgcgccgcccgggaggttgttgttgagctcgttggcagcggcggccgccggggtgcccagagcccccgcggggggcttcccagcggcgtcgctgctgccccctcccgggggggccgggcccggggggttctgcttggcgcgcatcttctcgcgtttcgccttccactcctccaggaagtctgtggtgctgccgccgaggccgctgctggtccggtagccaccggtcgccatattcccaaaggggccggtcgggctctcacctcaggccgcccaccagggctccggccgctgcctcctcttccttcctgcggccccgaggatgccaggagacgacctccaggagagggacggccgccgctcccacagcagccggcggggctacagtacggaccccgacgatcgcc

SEQ ID NO: 11179 - RNA, 8036 nt, Homo sapiens
  source 1..8036: mol_type = other RNA
ctgaatagctgggactacaggtgcatgccatcttgcccagctcatttatttttttgtatagacggcataaccctgtgttaccccgttggtattacaggcatgagccactgcacctagccaggcatattggttttaaaagggttacaagaaacaagatgcacttttaggcctcctataatcctgcatttccaaagcatccatttagtcatctcatcaaaattttcattgatttaaataagttaatatgaacagactgacataattttactttaatgatgttgtttattgtcctaagccatccatacacaaaacgtttaatgtgttatggaaggctaacagtttttcagcttttctcaatactttcagccatccatacataaaatgtttaatgtgttatggaaggctaacagtttttcaacttttctcaatactatcagatgaatgtattcttaccaatcatgatttacgtttttcaaatgtggatttcttaggcctttgactgatagctttaggcttttgcactacacaaagaaaaagacacctttctattcatttcttaataatttgtttccataaagctaaaatgtccactgatgacataatctacctttggttaatcacagcaaatagttcacattttaaaggaatgcagatatttggatagaagcctctaacaatgtaaatattgtgcatttcaagttccatagtgtgtctaaccagggatagcaactgattatatgtggattaacaatagtgaataactgagcacatattaacatgaataacatacacagcagtcaaaacttactgtttttcatatgtgtaaagtaaaaattcaatctatctttaaccggctcatactgttttcatgttgttcaactatttgacacaaaaggagctttttcctttctttaaaaggattttgattcagtcataacagatttttgaaagtgacagtaaaattatgcatttggtccaggattaagagggaagttttgcttgctagtgtctatctggttagacatcagaataaaatgaatggactgtaaaggatcttataaccagtctctctctttaatatgaaggcccaacattacataattctttttaagagttgaccaggaatgaaatgtaacctcttttaaagatgaagaaaaactgaaaaaatgagattaagaaaatatgtgggtagtttacagctgctgatagaattgtgtgcacgcgtgcatgcatgcataaacacaaagtgaatctagaagggaaaaaattgagtttgatgaagtctaagatgaaaggttccatttcatgtaagattatgtgaccttggaaaaatttactggcttgctagtggaatacgtccttatatagggacttgaagagtttatctaaatagactgacttaaggatgcttttcctcttgttagacttgtatgacattactgagaagatttagagttctagaagtagagaagactgattagcttgtgcctgtgtatgaagaatgacaaattaagacaaaaggttatgtaaaccatttactaaaaaagtctaaatttttatattcctaggcccctacttatcttttacaaactttgaaggacctgaaattctttggacaccatcagatttagtttataagagttctgattttgaatcaagaaattattcatgtagttttaaaacacaattaaaattttcagtcaggctgaacttttgtgcacttcctcatttattcgagaaaccccaccactaatgtatttagaccttaatatgatggctttgagtcttaaatcattgtccacctaaaataatataccaaataaagatttttaaagtgctgcatatggtttctgtaagaggtacataattagattaccagcattatcctttagcttcaaaagtaaaactcatagtcaggattttactgatagtacaggaagaaaaaaaataaccactgttgaaaaataaatgaaaaaaattttattgagtattactttatacatgcaaattgaaagtgaatctatattaagttgactattccacaataaaaacctatgaaatgggaatgatcaaagctgtctaacacaatactaatgtgttcaataaattatccagatgtttttccacaaatatttggattacctgaattagctgattcttcagcaaaagttaaattttagctttaatatggtagcagcaggatgctacttaaatttagaagaaaaacataagaataaaaaccctgaatagcatagccaaatcttccaagaaataagttcaccaaaaaagtagcatacacctatttggtatccagaggaggaaacaaaacacaggcacttaatcaacatccaccaagtgatcatcactaacattctattattaccagagtaactgtcgatatgtgaactgtagattagaacagacttacatatctaaaaacaaaccagtaatcaataatatatacagaaatactaacttgaagtcacatttaaataccatcaacagtttggtgtatctgatataactgaattcatttcatcactgctataaattccttaaaagtgttcttttcctaattaacattatctttaaaaaatggtagatatttcccagtatgcatcagttttttcactccaccattcagtaaatgttgtagcaaattaaatagaacctattaactagatctaaaaacagtggctgaatacttaacacaaagaagtacttttgagtaaactattcagattagacaggctaatgctaagactgcattttgtgctactgacatgcactatatagatcgtacactactagatggaaagttggtccatgtccatttatttaaagattctgtaacacctgtaatagtatttaatacagctcccacatactatattcctctcacatagacatagttatttttagtggggataaggatatgactttaacatgctatgagattctagctaagtaaaataaaaacaatatggactcagattttcttaggagatattagttcaagtttttaaactgggaaacaatcaacttccatatatccaggagaaacttagcatggggggaggtgccttagttgatgtgcctgataagcaaactgttagttgtctattagtattatgttttcggcttaatgtaacaacaaaagaaagttgtcacactacctctcagataatatcaattacaatcttagagactgtaattgggaatacaatcctataacaagttattaacaatatcatgaatagttattaagtaagtgccagcactacatgcaacttactggtcaccaactcagaacccataaaactatacacatatgcacaaaaaaaaaactccaaagaaagatacctatcactgtacatatgaatactgtccaggatatcagatcaattatcaaatccaaggtctctgctgttttgtcttacagtgttgaatatatgaatgcttctctattacactgacttgtactattttcaagaaattaagtggattcaaaatcttacatttttatttctaattataaaatccagattaatccaaaaaacacaaaccacatgtaaccgaggtaggtttttcaccttaagaatacattgcttctaccacaattaaaaattttttaaactgaagaaaaaaaaaaactacattgctccacatacctgatacttaattttctatgtttgaaactacttgaacaagtgtgacagtgctaatctactatatttagtaaatcccttagtacctataaatacacacccaaaagcccttccctccttctctaatggtaactgttgtataataaaattgtcaacaactctagaaagatgaaataaagattactatagcaatcttcaattaattcatttcagaaatcaaggaggcaagtcatgttcattttaaagatgacaaacttactattttgaaaatgagctcataaatacattagaactttgaatgtgctttattatgccacaaattcccaggagatttaagaaatagtatttctgaacaggaataataatttcacaaatactaacactttattgacaatagacaagtcttttagggtagtgcacatgtacttaaaaactaccttctaccaatctcaacactttttataaattttcaggtgaaactgtagcagatcctactttatttttcaatggttagtgtaaaattctgtatgtaaaataagtacatattttgagatggaagaaggactgcatgtgaaatgctttgcctaagttgtaaggctcctgtctttacgctatcattaaaggccaaaaaaatcactgctagaaatgttccccaaaaaattcttaaacagctcagtctttaaaagtattaataatttttttttttttttttttggagacagagtttcgctcttcttgcccaggctggagtacaatggcgcaatctcagctcaccgcaacctctgtctcctgggttttcaagcgattctcctgcctcagcctcctgagtagccaggattacaggcatgcgccaccacacctggctaattttgtatttttagtagagacggggtttctccatgttggtcaagctggtctcaaactcccgaactctggtaatccacccgccttggcctcccaaagtgctgggattacaggcatgagccactgcacccagcctaataactgatataatttttttaagtgaaatgaaatgttcctttatttacatatgaattaaatagaaaattcaaagtaattcttttaataaaaacccatatactaatatattttaaggttggatactaacagcattttcacaagatccaaagtgtggatgacgaactaggcaataaggacatgtgtgccacataactaagggtaactaaaggaagatgagtacctcacaaccaaaagcagttaactatgcctggcataccaccctgtcatgtgggcagatcactgttcccatgctgggtaagagtctccaagaagggaagcccttatgcagtaattctgtaactatattaaatttggtaatctaacattaaactttttcgtgagcagtgaatatacacatggtcatatgaaaactgccctggagaccgggttaattattaaataaactaaaaggggagaaatgctgatagataaaattatgtcaattccagggtgttcaatggaataaagaaacagcagcagctgcttcaaaagtagactatgatcagaaacctcagatggtaacctttaaaaattgtggaatccagagtctcaacctaaacctacataggagctacagccagggagttctttctaagttcctcaagtgattctgatgattggccaagctggaaacttctgaactgggggagaaagccaacctaggtaaatgtagagacttttagaattcaacatttgattatcatttactccacattttcccccagctgtctcaccttctctatttttctaacagtgaacaataaaagggcttggcaagtgaaggaaaaagtcagtagagtacctaaaatggatttgactatattcaagccactttcatatattaactagataaaaggataccatactgctatttgaaattcaatcacaaagcaaaaatgtcataattttaatgtattttaagggaagacggggttcttaacatgaatatgtaatacaaaaacaattctaaataataatatttaatagaagaaaaaatctgtataattatttagaagtaactctgtttttaaaatttcaatgttaggaagaaaatcccttaaatttgaaatagcggaatattctctcatatgaaaaaactgtgtcccagtgttattcttcaacttagaaattaggcaaagtattttagtactatttctgcttacatattgttttgtatgaatgttttaagtatgaataatattttggtttttagtgtgcatgctaatataaaaatatggatttttttctcctacactgactttgtacactttccaggcccgaagaataaaaaacttttaaaatatcctgtgttcactagcaaaccttggaacgataaaaaaaggtagtacctacataagaaattttacattgaaattacaattgtatgtttttcaggagttaaagtgattcaatttttcaatattcaaacacaaaatagtaaatttttatttactatagcacaattcaagtattctcttaaatttatatttagtcaactaaaacatgacagtgactttataagagctttccttttaaaaggttgctgttataaaaaagtatgactctattactctaaatgcttagaataagtggaaagaacaaatgacagtagacaaaaacctttatgagtgagtcatcaacacataaaaggttgcacacatcagtaataggacatgtgaaggtaacatcccaaaagtatttgaactcatgtaaacaaagactatgtatattcctaagggagaaaatgtactaccaagataaaatatattcaaacggctgtgactttaaaccatgtattagttgaataccacacaaaaccaaaaaggcattatctatcatttaataactgaaagatattacttatttgtgagataaaaggataatgcttttttaaaaccaataatgaaaaagaagtattttgaaaacaaacatctgtttgctagaaataaatatacttgcttagttattttaatgtattgcagcataggaatattgtgctagcattgaccattaacattcaatcagtagtttaaaatattttttccacattgagtcttgaatcctctacctggtcagctgacccacaactttcaaaagagttttattttcctgctttagctgttcattttcatcttctatgtcatctaggtctctatttaataaatcaatttcttctttgagttttccaatcatttcctctttatcttgcatcagtctcacaagtcttaggttttcttgtctttctcttactacttccttttcaagatcttcaattttcttttccagtgtgctacttgaaaccagagtacctgaaacatttgcatccctgttatatctagggaacccacttctatctgttcgagaatatctacttgagacatcttcttcagagacactggttgtgcttttatatctgcctgaaactgttctaggtggctcctgtagcagataggaactgcctggatctagtaagtttacagcttcattctgaatagtgttctgttgtgtaattgcatcttctcgtttccgctctttctgccctgcttcatcatcttcgtactcatctaagcactctgcggcagggatgttgaccacgccggtggagcgccgcttctcccgcagcttcctcttctcgatctgccccttgcctttcctggcactggggcccgagctcttgcccttctctgggacgccgtccggctcctcctcgtcacgctggggcggcggtgcagccgaggcagaggcggctgggggctcgtcctccgaccgccgcgggccgggggccgcccgcgtcagcatggcggagccgaccgcgcagttcacgcccccgggaccggggacggcaggtgcggccggcgcgccgcccgggaggttgttgttgagctcgttggcagcggcggccgccggggtgcccagagcccccgcggggggcttcccagcggcgtcgctgctgccccctcccgggggggccgggcccggggggttctgcttggcgcgcatcttctcgcgtttcgccttccactcctccaggaagtctgtggtgctgccgccgaggccgctgctggtccggtagccaccggtcgccatattcccaaaggggccggtcgggctctcacctcaggccgcccaccagggctccggccgctgcctcctcttccttcctgcggccccgaggatgccaggagacgacctccaggagagggacggccgccgctcccacagcagccggcggggcttggaggagcttgtaggggacgaggcgtagggctgggatccggctcccaggtgtgccgaagctggcgcgcgctcttccgccgcgcggaaagt

SEQ ID NO: 11180 - RNA, 5044 nt, Homo sapiens
  source 1..5044: mol_type = other RNA
ctgaatagctgggactacaggtgcatgccgacacgcctggctaatttttttgtattttagtagagatggagcttcaccgtgtttcccaggctggttgcgaactcctgagctcaggcaatccgcctgcctcagcctcccaaagtgctgggattacaagcgtgagccactgcgcccagccagaatttgaatcttaatacaagaactatgcaattttcagtggaaattttaagtcttgtagcagggctatggagtaagcattgtaaatatgatcaaagagatgaacacatcttgcataaagtatcaataatctgggtggtatattactgcttaaatggatggatcccagcaatatccattgcaataaaatttaaccaaaatgtttctggaagtttcttggccatctgttacaatagtatccaatctagagtatctataaaaaggaatgttactccctttcatgctttttttggcctcaaatgccagaacctttcgaatttgagaattttctgagtcttatcaaaaacaggatgaggagataaaaacagagttctgactctgtattcttttcagactctcagaaaagtgtctggattgaacacaaaaaatttaggcttatcaggtcactttattgcagcagtaacacttcattcagaaattagaaaggatttagtttgactagattaaagcacaaatttttatattagtatttttcattttctttgtgcattttaaacttttagaacttttcccacaaaaaacatagtactaaatatgcatttatggaatttagcatcttacgtttatactttttcttcttaattttatattattatagcagagtattctccgtatgagtctattacaatagaactttttcagtgttatagatccagtttgattcattccattaaactgaaaactacatatgtgaagtttaatatacaaacacatatgctgagatctaagttatatatacttgtcactgctgttttaatatggaaactaaccaagcaatttcttttagtttcagatgatcacttttttcctaaaatcagccaaattttgaaaagaaaaacactgtagaggtctttacagagtaaagttttcatttttaaattactttctgtaaaattggggagaaggtgttttgaggggagtctgtgctaaaacttaaaacaaaatttaacatttattttttgtttttgattttcttttacagacagggttctgctcagttgaacaggctagagtacagtggcatagctcactgcagcctccatctcaaggctcaagcaatccttccactacctcagcctctgagtagctggggctacaggtgggcaccatcatgcctggctaatttttaaattttttgtagacacagggtctcattatgttacccaagctggtcttgaacttctgggctcaagtgatccccctgccttggactaccaaagtgctaggattacaggcatgagccactatgcttggcctaatttttttttttatttttagtagagacaggatcttgctatgttgcccaggctggtctcaaactcctgggctcaagcaatcttccctcctcagcctcccaaagtgctgggattataggcgcaagccaccttacccagccaaaattaacatttataatagtgggtttgatgattggtcttagtagtatgttttgttgaacttctcaaaaatgagaaagtaacgttttatataactggacatgactgaatgaaatcattttctaaaagcttataataaggacatgaaagggtagtatggtcaaaatgtagattttttttcctgcaaaagaaccatccacaggcaaattatctaagtcccctgaatatgaaatatgacactattagaagtggtaaggtgcaactgcatgtatgacaaagtaagttgctgaatgtcttcacaatcaaaagcactaacttttaaaggcctcaagtactaaagcataattttagggatagaggaaagtgttcttgtttttgtaaatgagtatgggtcatggcatgactttggttttattttgggtcctcaaactgagagctttcttatgataatctgtatataaatagcaaaaaaaaacaatgggaatgttcataggataaataatatgagtgcaaatttttgccagaaagttctggaaatgtaggacttggttctttttataagtgcttttaaccttttcagactcattaatttcataaaccaatttaagcaattatttctatcagctacagatattttcttcacaaatataaagggttttgctcccctccccatcctccagcctccaccaatttgtgcctgtaactgccacttgatagctgctcagtaagactttaaatatcaggttctagtgccaacaaatccagaagtcagaaaaattctaagttacaatcgccagaatatctttcatgcattctattttactttattgttacagtttaaacaaattcagaaacgtggggtgtttctggctacttgagtaaaacgcactgcaaacgcaaagggaacaacgctgtaaacttaaatgatttctgaacagctcaggatcctcctggaggggatccttttcatctcacatattgattctgaacactatgttagcacctgctcccagaaggtcccttgacactggagcaagtcagaatatcttaatatcatagcttatttaacagcaggaaagcaactttaacatagacttgaggtttaggtagatctggtattatctagaacccaggcttaaattttgcaaaaagtttccaaagagcataagaaagtaaaacagaggtaccagaactgaagacatcattaacaaacaaaatatttccactcctaaccaaactgcaaccctttcagtatagcctgaggtatttttaaacatttgtacaagctaaagatcattcacagtttccaaagctgctttttactgagatagcttcaaattttcacaatatgtgactttcagacgttttcatataccagagtctctgccctcagactcatggaaacatcagagatatttagtggcagaaaatggttcttctagtgataagggttctatttcccaattattgtgctattcctaggatgtgattaaaaaaatatgaaatttgcaatttgtataaaaggaaaggaaacttgcttaaaattcaaaaagcaagtccagtctggtggaggtatgtaagatattaaataatagagtcagattctttcttgaacattccagatgaacttgacagcagagagttctggttttccaacattttctccatcttttcttttccagtggttttactgatctctctttgcttcttactatggatccacgggataaaacaaagcacagcacctccaataaggggagggactccagcgaggtagaatgccacatcataggagcccagtttgtcacgaagtaaccctgcaatgggtgggccaacagtcatgggtatagacatgaatccgagcagaaatccaattgcttgggagacatcctgggcaccaactaactcaaaggctatgggagccataatggaaatgaagcatccatcgaagagacccatgatgaggcacacagcaatgagggccccaaagatgctacacagaggaatcatcatggacatcagaccaatgaagaaaaaggagagtacctgtagataaaccttcttcacaccaggcacataatctgcaatccggccaaagagcagtcgtccaactcctgaagtgacgccaatgcacatgagaacaacctctttatttttttcatcttgaaatctttcatttacatgtttcatcaagtgaacataaggcacaaagtatccaaaaagtgcaagtggtattccaactgcccacactgcataagctgtcaccttgaagatggcaaaattgaaaattttttttggaggactgaactttttcctggaaaagagggaggatccgctacctccactctctttatctttggtactggtagcaagaggtcggtaagtaaagccagccagaaagagaacaaacatgaagatgcagagcaccctcaatgtgtaaaagaggcccacgctgtcaatcagaacccttaagagcaaaggcagcaggattgtgaagacactgctgccagcagtgacaatgccattcaccagtccaaggcgcttcttgaaatagtgtcccaaaatgaccaatgaaggctggtatgcaaaggagcagccgcaggcaaatatgattccataggtaaggtacagaggctcgatggaacaaacaaggtagtaaaagaaaaggccgcattttatattttttccccaaggttatgtcaggaacatttgcacagaggtgcagttgtgcctgtttttgctggcctaagggctgtagaccaaccttcgccctgtactgcactgttctcagtattgtgcaagacaacaagaaatcatattctgactacagaaagacttaaattaagtgtattcctttagtgatcccagtttgtaagctgtaaggccatgcatgtgtcaaaagaataatggattaaataatcttacagtttaaccaaataattgcacatttcttaggaagataaaggatcatatcattatgttctttgaaacaattatggtaaggaataaaactagttaaagttttttgaaaaggctatcagtagtaaaagcaaacaatttgttagaaagtaagattaaagttggttaataattaaaattttggataataatgctagtctagcaacatgctgaggtaatcataaggaactctagaatctgataaaattaaggcatgttggcaatcctctctctgagatgcccttctccctctactaatccacagctagcaccaccttcaaatcaggctcaagaatcacttctaggctttcccaaattaatctcacctcactctgatcaccctttactgaatctccactctttgtttagccaacatattaagcaactactgtgtaccagatacattgtggaaaagaatattaaaaatctggtccttggccagacgtggtggctca

SEQ ID NO: 11181 - RNA, 5013 nt, Homo sapiens
  source 1..5013: mol_type = other RNA
ctgaatagctgggactacaggtgcatgccgacacgcctggctaatttttttgtattttagtagagatggagcttcaccgtgtttcccaggctggttgcgaactcctgagctcaggcaatccgcctgcctcagcctcccaaagtgctgggattacaagcgtgagccactgcgcccagccagaatttgaatcttaatacaagaactatgcaattttcagtggaaattttaagtcttgtagcagggctatggagtaagcattgtaaatatgatcaaagagatgaacacatcttgcataaagtatcaataatctgggtggtatattactgcttaaatggatggatcccagcaatatccattgcaataaaatttaaccaaaatgtttctggaagtttcttggccatctgttacaatagtatccaatctagagtatctataaaaaggaatgttactccctttcatgctttttttggcctcaaatgccagaacctttcgaatttgagaattttctgagtcttatcaaaaacaggatgaggagataaaaacagagttctgactctgtattcttttcagactctcagaaaagtgtctggattgaacacaaaaaatttaggcttatcaggtcactttattgcagcagtaacacttcattcagaaattagaaaggatttagtttgactagattaaagcacaaatttttatattagtatttttcattttctttgtgcattttaaacttttagaacttttcccacaaaaaacatagtactaaatatgcatttatggaatttagcatcttacgtttatactttttcttcttaattttatattattatagcagagtattctccgtatgagtctattacaatagaactttttcagtgttatagatccagtttgattcattccattaaactgaaaactacatatgtgaagtttaatatacaaacacatatgctgagatctaagttatatatacttgtcactgctgttttaatatggaaactaaccaagcaatttcttttagtttcagatgatcacttttttcctaaaatcagccaaattttgaaaagaaaaacactgtagaggtctttacagagtaaagttttcatttttaaattactttctgtaaaattggggagaaggtgttttgaggggagtctgtgctaaaacttaaaacaaaatttaacatttattttttgtttttgattttcttttacagacagggttctgctcagttgaacaggctagagtacagtggcatagctcactgcagcctccatctcaaggctcaagcaatccttccactacctcagcctctgagtagctggggctacaggtgggcaccatcatgcctggctaatttttaaattttttgtagacacagggtctcattatgttacccaagctggtcttgaacttctgggctcaagtgatccccctgccttggactaccaaagtgctaggattacaggcatgagccactatgcttggcctaatttttttttttatttttagtagagacaggatcttgctatgttgcccaggctggtctcaaactcctgggctcaagcaatcttccctcctcagcctcccaaagtgctgggattataggcgcaagccaccttacccagccaaaattaacatttataatagtgggtttgatgattggtcttagtagtatgttttgttgaacttctcaaaaatgagaaagtaacgttttatataactggacatgactgaatgaaatcattttctaaaagcttataataaggacatgaaagggtagtatggtcaaaatgtagattttttttcctgcaaaagaaccatccacaggcaaattatctaagtcccctgaatatgaaatatgacactattagaagtggtaaggtgcaactgcatgtatgacaaagtaagttgctgaatgtcttcacaatcaaaagcactaacttttaaaggcctcaagtactaaagcataattttagggatagaggaaagtgttcttgtttttgtaaatgagtatgggtcatggcatgactttggttttattttgggtcctcaaactgagagctttcttatgataatctgtatataaatagcaaaaaaaaacaatgggaatgttcataggataaataatatgagtgcaaatttttgccagaaagttctggaaatgtaggacttggttctttttataagtgcttttaaccttttcagactcattaatttcataaaccaatttaagcaattatttctatcagctacagatattttcttcacaaatataaagggttttgctcccctccccatcctccagcctccaccaatttgtgcctgtaactgccacttgatagctgctcagtaagactttaaatatcaggttctagtgccaacaaatccagaagtcagaaaaattctaagttacaatcgccagaatatctttcatgcattctattttactttattgttacagtttaaacaaattcagaaacgtggggtgtttctggctacttgagtaaaacgcactgcaaacgcaaagggaacaacgctgtaaacttaaatgatttctgaacagctcaggatcctcctggaggggatccttttcatctcacatattgattctgaacactatgttagcacctgctcccagaaggtcccttgacactggagcaagtcagaatatcttaatatcatagcttatttaacagcaggaaagcaactttaacatagacttgaggtttaggtagatctggtattatctagaacccaggcttaaattttgcaaaaagtttccaaagagcataagaaagtaaaacagaggtaccagaactgaagacatcattaacaaacaaaatatttccactcctaaccaaactgcaaccctttcagtatagcctgaggtatttttaaacatttgtacaagctaaagatcattcacagtttccaaagctgctttttactgagatagcttcaaattttcacaatatgtgactttcagacgttttcatataccagagtctctgccctcagactcatggaaacatcagagatatttagtggcagaaaatggttcttctagtgataagggttctatttcccaattattgtgctattcctaggatgtgattaaaaaaatatgaaatttgcaatttgtataaaaggaaaggaaacttgcttaaaattcaaaaagcaagtccagtctggtggaggtatgtaagatattaaataatagagtcagattctttcttgaacattccagatgaacttgacagcagagagttctggttttccaacattttctccatcttttcttttccagtggttttactgatctctctttgcttcttactatggatccacgggataaaacaaagcacagcacctccaataaggggagggactccagcgaggtagaatgccacatcataggagcccagtttgtcacgaagtaaccctgcaatgggtgggccaacagtcatgggtatagacatgaatccgagcagaaatccaattgcttgggagacatcctgggcaccaactaactcaaaggctatgggagccataatggaaatgaagcatccatcgaagagacccatgatgaggcacacagcaatgagggccccaaagatgctacacagaggaatcatcatggacatcagaccaatgaagaaaaaggagagtacctgtagataaaccttcttcacaccaggcacataatctgcaatccggccaaagagcagtcgtccaactcctgaagtgacgccaatgcacatgagaacaacctctttatttttttcatcttgaaatctttcatttacatgtttcatcaagtgaacataaggcacaaagtatccaaaaagtgcaagtggtattccaactgcccacactgcataagctgtcaccttgaagatggcaaaattgaaaattttttttggaggactgaactttttcctggaaaagagggaggatccgctacctccactctctttatctttggtactggtagcaagaggtcggtaagtaaagccagccagaaagagaacaaacatgaagatgcagagcaccctcaatgtgtaaaagaggcccacgctgtcaatcagaacccttaagagcaaaggcagcaggattgtgaagacactgctgccagcagtgacaatgccattcaccagtccaaggcgcttcttgaaatagtgtcccaaaatgaccaatgaaggctggtatgcaaaggagcagccgcaggcaaatatgattccataggtaaggtacagaggctcgatggaacttacaaaagaactggacatgagcccaacaaatccaacagcagcacccacgacagctgttttccgacaaccaaataggtctgtgaagacgctgactattgggcagcaaaagaaaatcatccccatggagagagaacctacccatgctgtcttaaagaccatcttgtcatcgtctttggagccgaaggtttccagcatggacacgaagagcaccccgcaagcgttctggatgccgaacaccgacccgttgcaccacatggccgccagcatcaccagccagccccagccgccctcggggggttcggggggctcatggggctccgcggtcgccggccccgccagctccacctccaccttctcgacagccgcctcggggctgtccgagggtcccgggccgggcggcggagcggcccccgtgggcgcggggccgagcggctgcgcctcgctcgtgccccgcgcggagtccggctcctcctgggagagcaccatggcccgaggcgggcccctcaggcgccggagaagcgcgagggacgcgagttaccagcgggctcccggaggagctgcggggctcctggcgggctaacgaggccgaggcgagggcggcggagcccctggcgggcgggcgggctggcagcgcgcaggcggccagcgcgcaggcggccgcgaggacagctggcgcgcgcgaacacctcggggatcgacactgaagcctctaggtcacagccccgcacccccgact

SEQ ID NO: 11182 - RNA, 5045 nt, Homo sapiens
  source 1..5045: mol_type = other RNA
ctgaatagctgggactacaggtgcatgccgacacgcctggctaatttttttgtattttagtagagatggagcttcaccgtgtttcccaggctggttgcgaactcctgagctcaggcaatccgcctgcctcagcctcccaaagtgctgggattacaagcgtgagccactgcgcccagccagaatttgaatcttaatacaagaactatgcaattttcagtggaaattttaagtcttgtagcagggctatggagtaagcattgtaaatatgatcaaagagatgaacacatcttgcataaagtatcaataatctgggtggtatattactgcttaaatggatggatcccagcaatatccattgcaataaaatttaaccaaaatgtttctggaagtttcttggccatctgttacaatagtatccaatctagagtatctataaaaaggaatgttactccctttcatgctttttttggcctcaaatgccagaacctttcgaatttgagaattttctgagtcttatcaaaaacaggatgaggagataaaaacagagttctgactctgtattcttttcagactctcagaaaagtgtctggattgaacacaaaaaatttaggcttatcaggtcactttattgcagcagtaacacttcattcagaaattagaaaggatttagtttgactagattaaagcacaaatttttatattagtatttttcattttctttgtgcattttaaacttttagaacttttcccacaaaaaacatagtactaaatatgcatttatggaatttagcatcttacgtttatactttttcttcttaattttatattattatagcagagtattctccgtatgagtctattacaatagaactttttcagtgttatagatccagtttgattcattccattaaactgaaaactacatatgtgaagtttaatatacaaacacatatgctgagatctaagttatatatacttgtcactgctgttttaatatggaaactaaccaagcaatttcttttagtttcagatgatcacttttttcctaaaatcagccaaattttgaaaagaaaaacactgtagaggtctttacagagtaaagttttcatttttaaattactttctgtaaaattggggagaaggtgttttgaggggagtctgtgctaaaacttaaaacaaaatttaacatttattttttgtttttgattttcttttacagacagggttctgctcagttgaacaggctagagtacagtggcatagctcactgcagcctccatctcaaggctcaagcaatccttccactacctcagcctctgagtagctggggctacaggtgggcaccatcatgcctggctaatttttaaattttttgtagacacagggtctcattatgttacccaagctggtcttgaacttctgggctcaagtgatccccctgccttggactaccaaagtgctaggattacaggcatgagccactatgcttggcctaatttttttttttatttttagtagagacaggatcttgctatgttgcccaggctggtctcaaactcctgggctcaagcaatcttccctcctcagcctcccaaagtgctgggattataggcgcaagccaccttacccagccaaaattaacatttataatagtgggtttgatgattggtcttagtagtatgttttgttgaacttctcaaaaatgagaaagtaacgttttatataactggacatgactgaatgaaatcattttctaaaagcttataataaggacatgaaagggtagtatggtcaaaatgtagattttttttcctgcaaaagaaccatccacaggcaaattatctaagtcccctgaatatgaaatatgacactattagaagtggtaaggtgcaactgcatgtatgacaaagtaagttgctgaatgtcttcacaatcaaaagcactaacttttaaaggcctcaagtactaaagcataattttagggatagaggaaagtgttcttgtttttgtaaatgagtatgggtcatggcatgactttggttttattttgggtcctcaaactgagagctttcttatgataatctgtatataaatagcaaaaaaaaacaatgggaatgttcataggataaataatatgagtgcaaatttttgccagaaagttctggaaatgtaggacttggttctttttataagtgcttttaaccttttcagactcattaatttcataaaccaatttaagcaattatttctatcagctacagatattttcttcacaaatataaagggttttgctcccctccccatcctccagcctccaccaatttgtgcctgtaactgccacttgatagctgctcagtaagactttaaatatcaggttctagtgccaacaaatccagaagtcagaaaaattctaagttacaatcgccagaatatctttcatgcattctattttactttattgttacagtttaaacaaattcagaaacgtggggtgtttctggctacttgagtaaaacgcactgcaaacgcaaagggaacaacgctgtaaacttaaatgatttctgaacagctcaggatcctcctggaggggatccttttcatctcacatattgattctgaacactatgttagcacctgctcccagaaggtcccttgacactggagcaagtcagaatatcttaatatcatagcttatttaacagcaggaaagcaactttaacatagacttgaggtttaggtagatctggtattatctagaacccaggcttaaattttgcaaaaagtttccaaagagcataagaaagtaaaacagaggtaccagaactgaagacatcattaacaaacaaaatatttccactcctaaccaaactgcaaccctttcagtatagcctgaggtatttttaaacatttgtacaagctaaagatcattcacagtttccaaagctgctttttactgagatagcttcaaattttcacaatatgtgactttcagacgttttcatataccagagtctctgccctcagactcatggaaacatcagagatatttagtggcagaaaatggttcttctagtgataagggttctatttcccaattattgtgctattcctaggatgtgattaaaaaaatatgaaatttgcaatttgtataaaaggaaaggaaacttgcttaaaattcaaaaagcaagtccagtctggtggaggtatgtaagatattaaataatagagtcagattctttcttgaacattccagatgaacttgacagcagagagttctggttttccaacattttctccatcttttcttttccagtggttttactgatctctctttgcttcttactatggatccacgggataaaacaaagcacagcacctccaataaggggagggactccagcgaggtagaatgccacatcataggagcccagtttgtcacgaagtaaccctgcaatgggtgggccaacagtcatgggtatagacatgaatccgagcagaaatccaattgcttgggagacatcctgggcaccaactaactcaaaggctatgggagccataatggaaatgaagcatccatcgaagagacccatgatgaggcacacagcaatgagggccccaaagatgctacacagaggaatcatcatggacatcagaccaatgaagaaaaaggagagtacctgtagataaaccttcttcacaccaggcacataatctgcaatccggccaaagagcagtcgtccaactcctgaagtgacgccaatgcacatgagaacaacctctttatttttttcatcttgaaatctttcatttacatgtttcatctgaacagtcaaattgcagcagatgttgagatcaagtgaacataaggcacaaagtatccaaaaagtgcaagtggtattccaactgcccacactgcataagctgtcaccttgaagatggcaaaattgaaaattttttttggaggactgaactttttcctggaaaagagggaggatccgctacctccactctctttatctttggtactggtagcaagaggtcggtaagtaaagccagccagaaagagaacaaacatgaagatgcagagcaccctcaatgtgtaaaagaggcccacgctgtcaatcagaacccttaagagcaaaggcagcaggattgtgaagacactgctgccagcagtgacaatgccattcaccagtccaaggcgcttcttgaaatagtgtcccaaaatgaccaatgaaggctggtatgcaaaggagcagccgcaggcaaatatgattccataggtaaggtacagaggctcgatggaacttacaaaagaactggacatgagcccaacaaatccaacagcagcacccacgacagctgttttccgacaaccaaataggtctgtgaagacgctgactattgggcagcaaaagaaaatcatccccatggagagagaacctacccatgctgtcttaaagaccatcttgtcatcgtctttggagccgaaggtttccagcatggacacgaagagcaccccgcaagcgttctggatgccgaacaccgacccgttgcaccacatggccgccagcatcaccagccagccccagccgccctcggggggttcggggggctcatggggctccgcggtcgccggccccgccagctccacctccaccttctcgacagccgcctcggggctgtccgagggtcccgggccgggcggcggagcggcccccgtgggcgcggggccgagcggctgcgcctcgctcgtgccccgcgcggagtccggctcctcctgggagagcaccatggcccgaggcgggcccctcaggcgccggagaagcgcgagggacgcgagttaccagcgggctcccggaggagctgcggggctcctggcgggctaacgaggccgaggcgagggcggcggagcccctggcgggcgggcgggctggcagcgcgcaggcggccagcgcgcaggcggccgcgaggacagctggcgcgcgcgaacacctcggggatcgacactgaagcctctaggtcacagccccgcacccccgact

SEQ ID NO: 11183 - RNA, 3303 nt, Homo sapiens
  source 1..3303: mol_type = other RNA
ctgaatagctgggactacaggtgcatgccgccacacctggctacttttttgtattttagtagagacagggtttcaccgtgttgctcaggctagtctcgaactcctgagctcaggcagtctgcctgccttggcctcccaaagtgctaggattacaggcgaaagccaccgtggcccagccctggtatcttcttttatcttaggctctagactctgattcacagcctgaaccctatctcatgctgaaaacacctcccaccttcccaccaagagccttaacgtgggtcccacaccgctaagaccaagcaccttggatattggtatctatcttgatggaattttaggttgcctcatttctttttttcttgggccctggtggaaataaacctgagtgactgctccccagtgccatcacttgggcaggacactctgtcttagtttctccatgctgcctgtacaaggtcagtcccctatcccggctagcttggggcttcactgtggctgacaagagtattattactacctacacctcgtacagcacacaaccagaacctagagaaacttctttcaggcccactgatctataagcacaagcctccttagtgaactctgccctaaagtcctccttccagcatttggaagcattccaccatgaggagcaggtttaccttaagtctttgtccactttcagtttgcaataccactaggagagaaaaggtctggatgaagggatgaagatatcaggctgcaggtatttgaggtggctatgggggaagagaagagcaaaggagagggcaaaagaccaggctatggagaggcaggggagggaaaatcactgcttcactatttccattgggcctgacgctgagtggatcctggattgtttgcgtttgggaaggagggcccaaagggagaacagtaagcaagaaccaggttctccagagccctctccccagtctctggagagggtctgcagtgaaaggagctcgggtcttccctgagccaaggtgccagggtcccagaactgcacatgggcccacacccctctctgctacttcctcaggctcttgctcacaggcgtcgcatcaagcggccccgctgacgacggcgggcacctgggccacctcctggagtcatatcctggcgtaagatctgtagcagagaacgcaggttgcccagcactgagttatcattaggattctctgtaggaaagtcttctacaggtgggatggcaccctgggcaatgagctgcccgtaggaagggggtgcctgctgctgcacaatctcagcctccatccgggagaggggggcaaagatgctgtactcctgggtgcgaatggcatagagcttgcaggtgcagcccagggcgatgaccaggagcaggccgcacactaggctgccaatgactgcagctgtaatgaccttgcggggcagaacataggagcagtcccactcatcactgccgtccgcacagtctggctgcccatcgcacacccacgtctcatacacgcacttctcgtcccggcatcggaaattgccaggctggcaatgccgacagcgtctctcatctgctccatcagcacagaaagtctggtagttgcagcggtcagcaggcaggtagcaggctgtggcaccagaggtgccagcagccccacaggggaagtgtccaggtgggcagcctgggcagtcctcctcatctgtgccgtcagcacagtcccatgagccgtcacagcgctgtgcctcactgtagcagcgctcacctaggccttcgccagctcccaggccagagcctaagccacagggtctgtcccaaggcaagcaatagccccgcacatggtaggtggcattgaagccacgaccattgctccaagcaactgtgtggtaggacacaacagcctggccagacagtgtctccacagtgacagccttgccattgctgaagtgggtgagactacgcagtagtcgggagctctcagggggcccagggccgtcatacacatgcactgcatctccaaagcccaagtccagggctgtgaagcgcacggccagccgccggccatcatgggggtccagcagccaatggcaggactgggggtgggagactgaggctaggtgtgtatatccaggagaggagaagaccccatagaagtcctccaaggtgacattgcaaggcagggaggggacgggtcttggggtcaggccagggaaggggtctgagctgcaacctgcttcatcagagccatcgccacaggcatcaaccccatcacagcgctggacagcagatacacagcggtggttcaggcactgaaactcttcctgcaggcacatcagccaatcttggctgtaggagagcaggaagccctggcccatgggtgctctggccccagcatagctgtaagtgatggtgacgttgcccccgggcagctgcagagggctgggaggtgcctcacacagggagatcagtggctggagaggggagcgtagggttaagcgctctgagccacaggccaggtgtagcttctggaacctgatggtgacagtctgttccttgctgcccaggatgagccaggtgcagttggcaggggaggtgcggctgtcccggaccaggggcctctgtaaggtgccctgcacttctaagagcactgctggggggtcctcacaagcatgatttggaaaaataatccggtctggatgggccagagcgcctccaaggaggaggaggaggagggtggccaacagcatcctgggctgtccagaggtgccggaagggtcccggagcttctgtggtctacccgatggggtcgcggcggagccccgggcgcccaggctccctggtgccgcctccccaggggggctccatggcccgggctcgacccgtactctggatgccagggctgggggcggggaggcggcggcagcccgggagtaggggcggtgcctttcgccaactttggagttgttttctccgtccgccgccgcactcttctctcccggggccggctcctgaagccccgggtctcggcactggggcgcgccctcgcctacagcccgcccgcaggcagcgagcgcccctggtctggcctggtcgccacctgccggggtttgagaccacttcctcttcgggccaaactttgccgactgtcagcccccagggccggccgggtgctgctccactcctccagcgcgtccagccagcggagcgcgacagggaagcgggggaggggaagaggtggctcggcccggcgccccggcccttgcccaggcggtacccccgcccgcccaggggttggagtagccggggcgggt

SEQ ID NO: 11184 - RNA, 5599 nt, Homo sapiens
  source 1..5599: mol_type = other RNA
ctgaatagctgggactacaggtgcatgccgccacacctggctacttttttgtattttagtagagacagggtttcaccgtgttgctcaggctagtctcgaactcctgagctcaggcagtctgcctgccttggcctcccaaagtgctaggattacaggcgaaagccaccgtggcccagccctggtatcttcttttatcttaggctctagactctgattcacagcctgaaccctatctcatgctgaaaacacctcccaccttcccaccaagagccttaacgtgggtcccacaccgctaagaccaagcaccttggatattggtatctatcttgatggaattttaggttgcctcatttctttttttcttgggccctggtggaaataaacctgagtgactgctccccagtgccatcacttgggcaggacactctgtcttagtttctccatgctgcctgtacaaggtcagtcccctatcccggctagcttggggcttcactgtggctgacaagagtattattactacctacacctcgtacagcacacaaccagaacctagagaaacttctttcaggcccactgatctataagcacaagcctccttagtgaactctgccctaaagtcctccttccagcatttggaagcattccaccatgaggagcaggtttaccttaagtctttgtccactttcagtttgcaataccactaggagagaaaaggtctggatgaagggatgaagatatcaggctgcaggtatttgaggtggctatgggggaagagaagagcaaaggagagggcaaaagaccaggctatggagaggcaggggagggaaaatcactgcttcactatttccattgggcctgacgctgagtggatcctggattgtttgcgtttgggaaggagggcccaaagggagaacagtaagcaagaaccaggttctccagagccctctccccagtctctggagagggtctgcagtgaaaggagctcgggtcttccctgagccaaggtgccagggtcccagaactgcacatgggcccacacccctctctgctacttcctcaggctcttgctcactagaagagaggaaaattgtgcaattagtgctgggtttgaggaggctgacagggtgtaatcaacagggcctctccaccaggtgtggggctaggctgggtgatgggctctgccaggcgtggggctaggctgggtgacaggctctgccaggtgtggggctagacaaggagagcctgaggggagcctctttccccagggactgggtccgttagggaattcctcagttttgttcctgaggcatcactcccacccccacagcttccttctacatcttctgcctcgatcttccttccaaactctggggcagcttctgtcactttgctcactaggggctgggttccaacactgcttgcgaatcattccctccatcacccaccccagcgctgcagctctggccgctgcttgtgctctcaggcccagggtctttcctataacccttgccctcttgtctcctccgtttgcttgttctggggacactccccctgtctagaattcacagctctattccaactgctgacagcattcttttggttccagtttgggccctcttccaggaagacctcttggatttggccatggtgatgccagcaccacacaccctgaatgtttgtgaattctccctccactcacctttgcctgccttgaggtatcctggctgagaattcatctgtcttgcataggacagactgctaaatgcctggtgggtgtggagggtggagggtaggagtcatgactcctgtgtcccaccagggacagctgctcctatgatctgggctcagggtatgctccaaaaatgagaaccttcctgaccgcagggcccagctggctcccctgacttctatgctggcagtgaggaaagaggccctggagtcagtcattgcagagctgggccccaggcatttgagtgaaaatggagaggattgatccttagggttcctagaattttcttaccttctgtgtggtataaaaatcaagagtgcagtggttgggagatgaacaggaagagggcaggaggtagagggccaagcaaagggctccacagggaggagtgggatgaggtgagcatagactgagatgggcagaggcggggctcaggctcgcagctaatttgcaaaattttgagatgtatgattcctttatttttgacctcaacttactgagcaatgccgtagctatggaatagaagcatttgttgcactctttttgtgagccaggccctgtaggagggattgtggatggcaaaacctcaggttctgcccaaatcctccccttgggggctggagggtctctagttaattggcattccggtgcttaaggccacttttgggtagaggtttggcaaggatggagtgtccagacctatgatcctctaagaactttactttttaaaaacagccacccaaatggtggtggcgtggggagcaggtggtggtgaagggactggggtgtctggccatggccacgtacagaggagactctgtgagccctctccctgcctgagggacacttaactttatagcagctacatagggtcaacgggaggcccaccaagtccctgaaatccagggacagggaaggaagtggtggaggggaggctgacccacctctaaaaggttgtgccactatgagtagagcccccaggggagaggcctcagtagagcccccaggtcccctcaggtaagcagtggctcatcctctgcctcagctacccacacccccggctcagccagtggcaccagtagcacatcgtcctcatcttccagggccaggactgctgtgtggggtccaggggggctccgggttggtcctgggggccccaggctgggcaacaggcggcctcgcagggcctgcaccactccagacaatagtgatggctctaggggcagtgagggcagtggccctggggcttcagggacagtagtgggggctggagacgtgctagcagatgggaggggagccttgatgggcagtgggggtgcctgctccccatcttgcccacccactgccccgccctcacgggctggacctgtgccaccatctagggcctcaaggggagcagcagaaggtgtgacctgggatctggcctcagaggcccgagccggggtgttggttcgagggagcaagccccagcggcggagacggcgtaccaggcgtcgcatcaagcggccccgctgacgacggcgggcacctgggccacctcctggagtcatatcctggcgtaagatctgtagcagagaacgcaggttgcccagcactgagttatcattaggattctctgtaggaaagtcttctacaggtgggatggcaccctgggcaatgagctgcccgtaggaagggggtgcctgctgctgcacaatctcagcctccatccgggagaggggggcaaagatgctgtactcctgggtgcgaatggcatagagcttgcaggtgcagcccagggcgatgaccaggagcaggccgcacactaggctgccaatgactgcagctgtaatgaccttgcggggcagaacataggagcagtcccactcatcactgccgtccgcacagtctggctgcccatcgcacacccacgtctcatacacgcacttctcgtcccggcatcggaaattgccaggctggcaatgccgacagcgtctctcatctgctccatcagcacagaaagtctggtagttgcagcggtcagcaggcaggtagcaggctgtggcaccagaggtgccagcagccccacaggggaagtgtccaggtgggcagcctgggcagtcctcctcatctgtgccgtcagcacagtcccatgagccgtcacagcgctgtgcctcactgtagcagcgctcacctaggccttcgccagctcccaggccagagcctaagccacagggtctgtcccaaggcaagcaatagccccgcacatggtaggtggcattgaagccacgaccattgctccaagcaactgtgtggtaggacacaacagcctggccagacagtgtctccacagtgacagccttgccattgctgaagtgggtgagactacgcagtagtcgggagctctcagggggcccagggccgtcatacacatgcactgcatctccaaagcccaagtccagggctgtgaagcgcacggccagccgccggccatcatgggggtccagcagccaatggcaggactgggggtgggagactgaggctaggtgtgtatatccaggagaggagaagaccccatagaagtcctccaaggtgacattgcaaggcagggaggggacgggtcttggggtcaggccagggaaggggtctgagctgcaacctgcttcatcagagccatcgccacaggcatcaaccccatcacagcgctggacagcagatacacagcggtggttcaggcactgaaactcttcctgcaggcacatcagccaatctgcagaggcaccatggagaggggcttggctgtaggagagcaggaagccctggcccatgggtgctctggccccagcatagctgtaagtgatggtgacgttgcccccgggcagctgcagagggctgggaggtgcctcacacagggagatcagtggctggagaggggagcgtagggttaagcgctctgagccacaggccaggtgtagcttctggaacctgatggtgacagtctgttccttgctgcccaggatgagccaggtgcagttggcaggggaggtgcggctgtcccggaccaggggcctctgtaaggtgccctgcacttctaagagcactgctggggggtcctcacaagcatgatttggaaaaataatccggtctggatgggccagagcgcctccaaggaggaggaggaggagggtggccaacagcatcctgggctgtccagaggtgccggaagggtcccggagcttctgtggtctacccgatggggtcgcggcggagccccgggcgcccaggctccctggtgccgcctccccaggggggctccatggcccgggctcgacccgtactctggatgccagggctgggggcggggaggcggcggcagcccgggagtaggggcggtgcctttcgccaactttggagttgttttctccgtccgccgccgcactcttctctcccggggccggctcctgaagccccgggtctcggcactggggcgcgccctcgcctacagcccgcccgcaggcagcgagcgcccctggtctggcctggtcgccacctgccggggtttgagaccacttcctcttcgggccaaactttgccgactgtcagcccccagggccggccgggtgctgctccactcctccagcgcgtccagccagcggagcgcgacagggaagcgggggaggggaagaggtggctcggcccggcgccccggcccttgcccaggcggtacccccgcccgcccaggggttggagtagccggggcgggtgacaagcccggtcccacccctgccaatcaacgcacgggccacacccacttgctcgccttaacccctttcccggccctgccggacttgtcagacgggcccttgacttgcagcttcagcttccacattt

SEQ ID NO: 11185 - RNA, 5448 nt, Homo sapiens
  source 1..5448: mol_type = other RNA
ctgaatagctgggactacaggtgcatgccgccacacctggctacttttttgtattttagtagagacagggtttcaccgtgttgctcaggctagtctcgaactcctgagctcaggcagtctgcctgccttggcctcccaaagtgctaggattacaggcgaaagccaccgtggcccagccctggtatcttcttttatcttaggctctagactctgattcacagcctgaaccctatctcatgctgaaaacacctcccaccttcccaccaagagccttaacgtgggtcccacaccgctaagaccaagcaccttggatattggtatctatcttgatggaattttaggttgcctcatttctttttttcttgggccctggtggaaataaacctgagtgactgctccccagtgccatcacttgggcaggacactctgtcttagtttctccatgctgcctgtacaaggtcagtcccctatcccggctagcttggggcttcactgtggctgacaagagtattattactacctacacctcgtacagcacacaaccagaacctagagaaacttctttcaggcccactgatctataagcacaagcctccttagtgaactctgccctaaagtcctccttccagcatttggaagcattccaccatgaggagcaggtttaccttaagtctttgtccactttcagtttgcaataccactaggagagaaaaggtctggatgaagggatgaagatatcaggctgcaggtatttgaggtggctatgggggaagagaagagcaaaggagagggcaaaagaccaggctatggagaggcaggggagggaaaatcactgcttcactatttccattgggcctgacgctgagtggatcctggattgtttgcgtttgggaaggagggcccaaagggagaacagtaagcaagaaccaggttctccagagccctctccccagtctctggagagggtctgcagtgaaaggagctcgggtcttccctgagccaaggtgccagggtcccagaactgcacatgggcccacacccctctctgctacttcctcaggctcttgctcactagaagagaggaaaattgtgcaattagtgctgggtttgaggaggctgacagggtgtaatcaacagggcctctccaccaggtgtggggctaggctgggtgatgggctctgccaggcgtggggctaggctgggtgacaggctctgccaggtgtggggctagacaaggagagcctgaggggagcctctttccccagggactgggtccgttagggaattcctcagttttgttcctgaggcatcactcccacccccacagcttccttctacatcttctgcctcgatcttccttccaaactctggggcagcttctgtcactttgctcactaggggctgggttccaacactgcttgcgaatcattccctccatcacccaccccagcgctgcagctctggccgctgcttgtgctctcaggcccagggtctttcctataacccttgccctcttgtctcctccgtttgcttgttctggggacactccccctgtctagaattcacagctctattccaactgctgacagcattcttttggttccagtttgggccctcttccaggaagacctcttggatttggccatggtgatgccagcaccacacaccctgaatgtttgtgaattctccctccactcacctttgcctgccttgaggtatcctggctgagaattcatctgtcttgcataggacagactgctaaatgcctggtgggtgtggagggtggagggtaggagtcatgactcctgtgtcccaccagggacagctgctcctatgatctgggctcagggtatgctccaaaaatgagaaccttcctgaccgcagggcccagctggctcccctgacttctatgctggcagtgaggaaagaggccctggagtcagtcattgcagagctgggccccaggcatttgagtgaaaatggagaggattgatccttagggttcctagaattttcttaccttctgtgtggtataaaaatcaagagtgcagtggttgggagatgaacaggaagagggcaggaggtagagggccaagcaaagggctccacagggaggagtgggatgaggtgagcatagactgagatgggcagaggcggggctcaggctcgcagctaatttgcaaaattttgagatgtatgattcctttatttttgacctcaacttactgagcaatgccgtagctatggaatagaagcatttgttgcactctttttgtgagccaggccctgtaggagggattgtggatggcaaaacctcaggttctgcccaaatcctccccttgggggctggagggtctctagttaattggcattccggtgcttaaggccacttttgggtagaggtttggcaaggatggagtgtccagacctatgatcctctaagaactttactttttaaaaacagccacccaaatggtggtggcgtggggagcaggtggtggtgaagggactggggtgtctggccatggccacgtacagaggagactctgtgagccctctccctgcctgagggacacttaactttatagcagctacatagggtcaacgggaggcccaccaagtccctgaaatccagggacagggaaggaagtggtggaggggaggctgacccacctctaaaaggttgtgccactatgagtagagcccccaggggagaggcctcagtagagcccccaggtcccctcaggtaagcagtggctcatcctctgcctcagctacccacacccccggctcagccagtggcaccagtagcacatcgtcctcatcttccagggccaggactgctgtgtggggtccaggggggctccgggttggtcctgggggccccaggctgggcaacaggcggcctcgcagggcctgcaccactccagacaatagtgatggctctaggggcagtgagggcagtggccctggggcttcagggacagtagtgggggctggagacgtgctagcagatgggaggggagccttgatgggcagtgggggtgcctgctccccatcttgcccacccactgccccgccctcacgggctggacctgtgccaccatctagggcctcaaggggagcagcagaaggtgtgacctgggatctggcctcagaggcccgagccggggtgttggttcgagggagcaagccccagcggcggagacggcgtaccaggcgtcgcatcaagcggccccgctgacgacggcgggcacctgggccacctcctggagtcatatcctggcgtaagatctgtagcagagaacgcaggttgcccagcactgagttatcattaggattctctgtaggaaagtcttctacaggtgggatggcaccctgggcaatgagctgcccgtaggaagggggtgcctgctgctgcacaatctcagcctccatccgggagaggggggcaaagatgctgtactcctgggtgcgaatggcatagagcttgcaggtgcagcccagggcgatgaccaggagcaggccgcacactaggctgccaatgactgcagctgtaatgaccttgcggggcagaacataggagcagtcccactcatcactgccgtccgcacagtctggctgcccatcgcacacccacgtctcatacacgcacttctcgtcccggcatcggaaattgccaggctggcaatgccgacagcgtctctcatctgctccatcagcacagaaagtctggtagttgcagcggtcagcaggcaggtagcaggctgtggcaccagaggtgccagcagccccacaggggaagtgtccaggtgggcagcctgggcagtcctcctcatctgtgccgtcagcacagtcccatgagccgtcacagcgctgtgcctcactgtagcagcgctcacctaggccttcgccagctcccaggccagagcctaagccacagggtctgtcccaaggcaagcaatagccccgcacatggtaggtggcattgaagccacgaccattgctccaagcaactgtgtggtaggacacaacagcctggccagacagtgtctccacagtgacagccttgccattgctgaagtgggtgagactacgcagtagtcgggagctctcagggggcccagggccgtcatacacatgcactgcatctccaaagcccaagtccagggctgtgaagcgcacggccagccgccggccatcatgggggtccagcagccaatggcaggactgggggtgggagactgaggctaggtgtgtatatccaggagaggagaagaccccatagaagtcctccaaggtgacattgcaaggcagggaggggacgggtcttggggtcaggccagggaaggggtctgagctgcaacctgcttcatcagagccatcgccacaggcatcaaccccatcacagcgctggacagcagatacacagcggtggttcaggcactgaaactcttcctgcaggcacatcagccaatcttggctgtaggagagcaggaagccctggcccatgggtgctctggccccagcatagctgtaagtgatggtgacgttgcccccgggcagctgcagagggctgggaggtgcctcacacagggagatcagtggctggagaggggagcgtagggttaagcgctctgagccacaggccaggtgtagcttctggaacctgatggtgacagtctgttccttgctgcccaggatgagccaggtgcagttggcaggggaggtgcggctgtcccggaccaggggcctctgtaaggtgccctgcacttctaagagcactgctggggggtcctcacaagcatgatttggaaaaataatccggtctggatgggccagagcgcctccaaggaggaggaggaggagggtggccaacagcatcctgggctgtccagaggtgccggaagggtcccggagcttctgtggtctacccgatggggtcgcggcggagccccgggcgcccaggctccctggtgccgcctccccaggggggctccatggcccgggctcgacccgtactctggatgccagggctgggggcggggaggcggcggcagcccgggagtaggggcggtgcctttcgccaactttggagttgttttctccgtccgccgccgcactcttctctcccggggccggctcctgaagccccgggtctcggcactggggcgcgccctcgcctacagcccgcccgcaggcagcgagcgcccctggtctggcctggtcgccacctgccggggtttgagaccacttcctcttcgggccaaactttgccgactgtcagcccccagggccggccgggtgctgctccactcctccagcgcgtccagccagcggagcgcgacagggaagcgggggaggggaagaggtggctcggcccggcgccccggcccttgcccaggcggtacccccgcccgcccaggggttggagtagccggggcgggt

SEQ ID NO: 11186 - RNA, 1423 nt, Homo sapiens
  source 1..1423: mol_type = other RNA
ctgaatagctgggactacaggtgcatgccgccatgcagctaatttttaaattttttttgtaaagacaggatctcactatgttgcccaggctggtctcaaactcctggactcaagtgatcttcccgccttggcctcccaaaatgctaggattacaggcattagtcaccagtcccagcctgaaatgtacttaaagttattagcatacataatataccctcaaatattgttcccttttccttttttttttttttttttttttttcgagacagggtcttgctctgtcacccaggctagagtgcagtagtgcaatcatagctcactgcagactcgaaattctagattcaaatgaccctcttgagtaactagaactacagatgtgggcacccacaacctgctaattttttaatttttttgtaaagagggggtctcactatgttgcccaggctggtccctttttccttcttactagaaaatttctagctcccttccaagaatctcagcttatacctggttctttcaatatgtggttaataactgtcaactaaggactgaaagtattttcaatccttgagccatgcctatggctcttcatctgggggacagaactctttaactgagtataatgaacacctcatagattacattttctaggcaaaatttttaaccaatgccaacaatgtccacagagaaaaattagattgaattaacttttattactacttgtttaacacagatttacttgtcttagacaagtaagaatttatagaatctatgctctattgcactatatagaaactagaaatgcagttatactgatgtagtgcagtttgtgggaaatcaggaatggtgttctccagaatacatgaagattctcattgattgttgcaaggaatcacgaaagagatctttggtccaaagaaaacgtcttttgggcagcagagcaattcgctgaagttgcagtaacagatcatctcacatcccttcccatcccagaaatgatcctggacattgacatcaatctgtgtcaggtcagctactccttccggaaggttgtgacagttgtgatcttttagtatctttctgtagcaagagaggcgatttgcaggcatggcttgaactcctagcagcaaagttagcccaatggtgaaaacaagtaccatcagtttcattttggcttttggccctttgtgcacatcgggcaagtggttcgtcttcccaggtatgaagggagtgtcatttccttttctccaaaacttccgggttgccttcggggcccttcggtgctgtgtagtcggcgtggcgctgtgagctaggcgaacaggaacccccaggcccgccacgtctacgctattagcagccaggtagccctgcgggtcgaagatgctcagaggaggagtaaatgcagagaaaaaatagaggaagg

SEQ ID NO: 11187 - RNA, 1232 nt, Homo sapiens
  source 1..1232: mol_type = other RNA
ctgaatagctgggactacaggtgcatgccgccatgcagctaatttttaaattttttttgtaaagacaggatctcactatgttgcccaggctggtctcaaactcctggactcaagtgatcttcccgccttggcctcccaaaatgctaggattacaggcattagtcaccagtcccagcctgaaatgtacttaaagttattagcatacataatataccctcaaatattgttcccttttccttttttttttttttttttttttttcgagacagggtcttgctctgtcacccaggctagagtgcagtagtgcaatcatagctcactgcagactcgaaattctagattcaaatgaccctcttgagtaactagaactacagatgtgggcacccacaacctgctaattttttaatttttttgtaaagagggggtctcactatgttgcccaggctggtccctttttccttcttactagaaaatttctagctcccttccaagaatctcagcttatacctggttctttcaatatgtggttaataactgtcaactaaggactgaaagtattttcaatccttgagccatgcctatggctcttcatctgggggacagaactctttaactgagtataatgaacacctcatagattacattttctaggcaaaatttttaaccaatgccaacaatgtccacagagaaaaattagattgaattaacttttattactacttgtttaacacagatttacttgtcttagacaagtaagaatttatagaatctatgctctattgcactatatagaaactagaaatgcagttatactgatgtagtgcagtttgtgggaaatcaggaatggtgttctccagaatacatgaagattctcattgattgttgcaaggaatcacgaaagagatctttggtccaaagaaaacgtcttttgggcagcagagcaattcgctgaagttgcagtaacagatcatctcacatcccttcccatcccagaaatgatcctggacattgacatcaatctgtgtcaggtcagctactccttccggaaggttgtgacagttgtgatcttttagtatctttctgtagcaagagaggcgatttgcaggcatggcttgaactcctagcagcaaagttagcccaatggtgaaaacaagtaccatcagtttcattttggcttttggccctttttcttctttccttttggtcttggcagaggatgcttcttaaatgct

SEQ ID NO: 11188 - RNA, 5965 nt, Homo sapiens
  source 1..5965: mol_type = other RNA
ctgaatagctgggactacaggtgcatgcgacccagcccagctcagtatggttttaatggtaaatatttcactaagccagtacttattttttacacagtagttggtaattcacagaaggtagcaaacagaccacttgtaacaatccaagatacagttttactgagcttatattcatatactgaataataattattaagctatatacttacagaaaagaggatatgaaaatattaatcaagtatgacctctactggtaacttttatgcactgtcaacaagagatctaagatttttattgagctcctaccataaagacacatcatttcaattcaaccatcagtagcctctactttttaaaaaaatatttttatttttttagtggcttgaaacagcaacagtcattattatctctcatggttcatgtgggttggtgtttgggaagtattcagtggggtggttctgggttggggtgtcccgtgatgttgcagtccgatggtagctggaactgcagtcatctcacgagcttcttcattcacatgtctggtacccgcgcaggatgatccaaatatctggagtctgaaacagctggggctcctgggtgcctccctctatctctgtgtgatgtctctacatggtctcttctgcatgacggcttcatggtagctggacttcttacatggtggctcagggtgtcaaagacacatgtcccaggagagaaagacagaaccctaggctgaaggaatattacctttttctaactcagaaatcacagtgtcactttgccgattcgttataagtatatatctaagatcaacccacactggaaggaaatgacagcctctattttaaaattaccttgttggaggctctcagattaggacagtagtgatgttgaacatgcatctgaatatctcttggaaatgtcaattctgcccatgcaatgtctgtaatcaagccatgacttactctgctgtcaatgttctctctcacacatttgaagacgcaatgggaggggctgctacattgaacagaattctgaacagcaaggacctacttggtattctggaaagtatggggcaacttggggcgtgatgtcagccagagtccttccaccaaggcttttatggtgttacgtgatccaccaccccattaacactctgatctaatctccagcccctctccctgttgttcactgcactccagctacactggcctccttgggtcaagcacaccaagcacattactgtttcggaacctccacacgtgctgctcctttgcttcgacctctcgtctcccacatatccacctaattccctctgctcctttcacgtttcagcttaaatgtcaccaaggcctctcctgacacatctttatattagaacaacctaacaatacgttctttatcccctttactctgctgtttctccacagcacttattactacttaatataaggacatagtgtttattgttacagtttgtctctttgaattggaatgtaaattccaaggcagggaatttgattatattgttaatcacagtgctcaataaatagttgttgtacaagcaaatgaattaatgtaggagaaaggaattgtgtcacttaggatttattataacactaacaacaataacagagaaaatatacactgatacgacttataagacattacattcttttatctttggatttatttttttaatctaaggaatgaagactttgaaattcagttaggaggtccaaaaggtgggaaagggaaaggcttaggaagttctaaaacatgatatgtgagtagtatgattattaattatcttaatgaagaagaaaacagaaaaactgttaaagaactcaatgtggctaaggagaaagattgctcagaaaaaaagtgtacacacacaaacagcagatgcagagaggaacacacagagaggagtggaaatgtgcagctggagcctctaaaagtgccccaaacaagccaaacacacacaccacctagaccaagaaaagacataagaccaactaatgcatatcccaagaggcattccaaggagaaagaaaaaggaagtgttaagcctacgaattaatcagactggtagaggacgaaaaagcagaacaattctccatatcagaaaactaatatacaaacaggaaaggtcaacaaatacaacccccatggcttttttaatgttgataagaagtaagtccagaattctcattttatttctcatccttgagagaaaacattttccacaaggcaggtcaagattttatatgtttatttgtggttagaaggaaacgaaaactaataagaaagaacatagttaagagagagctgaacatgaaatgggtttattattgtcatttgaaaaggaactaataagtaaatattgttttacttatttctcagttttaatttctgatatggtaagcattaatacaatccacataagcaagaattcttcggagtcctcaataagtttttagagtttcagggggtcatgagactgaaagttgacaaccaccgtccttaaataaagacaactttacacccaccctaacaaacattaaaaacaaacaagattccaaaggatcaagtcgacccaatagtaactcaactgcctgccaaaacacacctcaatgctctttgaactttaggacaaggaatattatcagcgataaagatggagatttcataatgatgaaagaattatgtcattaaaaatacataataatccttagcatatttgcatataattatacagcttcaaaatacatgaagcaaacctgacagaactaaaaagagaaacaaaaaactataattatatttggagatttcaacaatcatctctcacttgttgataggacaaagaccaaaaaaaaaaaaaatcagcaagtatacagaagacttgaaaaaaactgtcaaccgatttgacctatcatttatagagtaatattccccaaaatagcagaatgtacattattttcaaatatacaaggatcatttaccaagataaaccataattttgggccataaaacatttaggattgaaaatacagagcaaattctctaaccacaataaatttaaaaaatcgatagccaaaagataactgaaaactcccccaaatgtttgaaaattaacacatttctagaaaagtcatagatcaaaattaaattacaagggaaatctgacactattttgaactacgcgttcatgaaaacacatcaaaacttgtgaaatgcagctaaaacagtgcttggagagagaaaagttctaaaattactaatataaacttctaccttaaaaaagctagaagaaaagcaaactcaaagtagaaggaaagaaataaagataactgcagaaatcaatgcgatagaaaataagcaaatagagaaaattagtaaaaccaaaagttgctcctttaaatgatcaataaaaattacaaacccctaactaaagcaatgaacaaaagagaagatataaattaacaatattaagaacaaaagaggacaagtgactatggcttttgtagccattaaaaggatatcaagggaatactgtcaataactttataccaataaattcaacatttagatggaatggacaaattccttgaaaggcacaaattaccaaaactgaaacaagaagaaatagaaaatatgaatattaaagaaattaaattcaaatttcaaaattttcccacaaacagaactctagccccagataacttcagtgatgaatcatatcaaacatttagggaaaagattattccaaactcatacagatactgggccagtcaaaaaaggaattctgttatgcaaagcagcaaattcccagtactggaaatacagtttctggcattcctccactgggaagaaatctaaatcttcacttccaaacgcacactgtagattcttttcactagatatgccacacaggtaatggcccaaagtctcattatcatccttctcttttcaaactggagttgaaaatgtgtcagctctggatcagattaatatcatgtccatctttccaaacttaaacccatccatcagggtcattccagaagctagagggcattttccaaagattcaacacctacaactcaattgcattctgggtatataattcatattttatccccattgtataactggagcttcataactttctttaatcatgttatagtctctaaggttggagttactgttacacttgtcataaggtaaccctaaaaacgagattttaaaaaatatacctagttgacttaagaaatgatcccagagagactgccaaaagtacacatccacacattaaattttctttataatgatctttatggaatatttgtttatttgacattaaattggaagtttgagcaaaaacactgtaagaagttgttttcccagtcttaaagctgattctactggtctaatgtggtatttctcataatctacatttaggccactgaacagtgaaaaacaagttgaatctttaaaacagcagaaattctctggttagagactatggagcctcatttacttgtccatttctctcaacaaattcacatgacccccaagatactttctcaaaatctctagggttctctggaacactatttataaactaactatttgcctggcttatctgcagtgttaaccctacaaagtcatgtaaatcagcactagaggaaaatttaacttaccaatcgggctatagacaccctgaatgttggacatgccatatggaatcggggaatggcaacattaaagatcttgtctttaaagtaaagaaaatggaaggtataatatccttccatgtatcctgatgttgtagagaatgtggtacagcttgtgtattcatatacccgacctgggctgatgattggaaattcaccaactactccaggtccttgaacttcttccacgtcacccttagcatttgttattctccaatagcgactgtccaactgacaggccttctcaggaagtgcatcttttgacatttcaatcctgattcggtatgtgaagaaatagtggggtggatgtacagagctaagttctggcagaaacgatgtggaaactgacacagtaatatccccagttgttgctacacattctggatcgtgaacatatctgaaaatttggtctctgatgatggggaagccacctgatacaacatttttgacataagaggtaaaccagtcagtaaaagtagcacctataataaacatgtcaatagcagctggatttcgagccatttggtctggacattggtagaaaacttcatttttgtttcggccctctgcagcttccactgctatgtactgactcaaaccagtatgtatgcaaaaagttaaagggagacagtatttcagtccctgtctctgctggaatcctccggcagctgtatcgacgtctaacaaatcttcagaacgatagtgattagacagtgccatgcttcccaataacccaggaaccactaacttctgtccattgtgaattcggtatgaacatcgataatcgtcaggaagcttgcagccaatctgcgcttccacagcatcgaggtcttcctctcgagcaccctctttcagagataaaaccatccgaggacacctgggctccaaatatttcttgagatcatcccaggcctttttaatagcagcataatggtcaatgtatcttcctacatcagagtaagtatctatgaagagagatttccaacactgattcttctgtgttttctcttcctcagatatcagccagtattttttgcaatgtcttctccacagcggatcatgacttgatagctggctaagtcttcgactgacataacaacagttgattagatcccgatagtccaaaaaggataagatgaggagcaggggatcggtgggcagcgactctagggtcagcggcgccgtctcggtctccatggccgccatcttgcctggcccggtgcaggtct

SEQ ID NO: 11189 - RNA, 5717 nt, Homo sapiens
  source 1..5717: mol_type = other RNA
ctgaatagctgggactacaggtgccaccacgcccggctaatttttcaatcttttttttttttggtagagatggaatctttctatgttgcccaggttggtcccaacctcctggcctcaagcaatcctcctgccaaagtactgggattacaggtgtgaaccatctcatccagcccaaaattctttctcaagcaaaggcgccttgcccagaggggaaaatgcagatgttttattccctccctctcctcaggcatcaggtattctgccattttgaggcacctggctcccttacctcagatccttttccaggttattctttttgccttcttgcctatttcctgccaaaccatatcctgtttttgtttttgtttttgtatcgagacgagtctcactctgtctcccaggctggagtgcagtggcgcaatctcgactcactgtaagctctgcctcccgggtgcaagtcattctcctgcctcagtctcccaagtagctgggactataggcacctgtcaccatgcccggctaatatatatatatatatatatatatattttgtatttttagtagacacggggtttcactgtggtagccaggatggtcggtctcaatctcctgacctcgtgatccgcccatttcggcctcccaaagtgctgggattacaggcatgagccaccgtgcccgattgtttttgttttatgaaattttattctaatctcacatcttctaggcattctgctgggtttacactggcagattctggagactccgttccatcttcaggtagtcataggggtaacctctcacatggccatgactataacctttactattttgaaaatattctagcatttgttcccagaacaactctgtgggagtagatactgttagtcccatatgagcaatctaaggctcagcatcagtgacttacccaacaccacccagctaataagacgccgagccccaaattgaatccagacccgctggctcccactccagtgctctttctactgttgtgaaacccagacccctcaactatcacccttattactaagcactcatttgtgttgatgcagttgttcttgttatttgttcttgttatcctgcaccttcatgttcttgtcaattgtatttgtagccacgtgcttactatgtttccttcctgtgattgggaacttccagaggtgagggatggaattttcctttctctgttggtccctcagaacccaggataggggtctgccaaccaaaggaacggaccctgaggataaaggcaggcaccatggttgtggatctttgccaccttcaagtgcatatggagagtggatgtggacagaaatttgataacagtaagtaacagcagctgctatttgttgagcacttactagatgctgagtgttatgctagttctttatttacattatttaatcctcacaacaaacttctaagggaggtattattattggcaaatgagaaatctaatgctcagagacatggagttaggatgcaaccacatctgtctgactccaaaaggatcacataaatagtagaattcaatttaaaaaatatgtaccgggcgtggtggctcacacctgtaatcccagcactttgggaggccgaggcaggtcgattacctgaggtcaggagttcaagagcagcctggccaacatggtgaaaccctgtctctactaaaaatacaaaaattagttgggcgtggccaggcacggtggctcacgcctgtaatcccagcactttgggagatgaaggcgagtggatcacctaaggtcaggagttcgagaccagcctggccaacatggtgaaaccccgtctctactaaaaatacaaaaattagccgggcgtggtggtaggtgcctataatctcagctactcgggaggctgaggcaggagaattgctggaacccaggtggcgaaggttgcagtgagctgaaatcattccagccctggtgacaatagcgagactctgtctccaaacaaaacaaaacaaaaattagccgggcgtggtggcaggagcctgtaatcccagctactcaggaggctgaggcatgagaatcacttgaacccgggaggcggaggatgcagtgagccgagattgtgccattgcactccagcctgggcgacagagcgagattctgtctcaaaaaaaaaaaagaaagaaagaaagaaaaaaaaaaaaagataatccctcactccctgaaggcccaccctacccttgacttttcttttcccaaaaaataaaattcaggaagaggaaagcagaacaggttgtacctcatacataagcacacacacattttcacacacacacacacgcatacacacaccacttatacctatcaccaccaccctggatttcctagccccagggtgagggctatgaggggtcaggggtcaggttccccaggaccctagtccttgtccccttccctggtgctaaataaaagtgaataaatactaaataaatacaactggggcccaggccctccctgccttccccctccctcctgtgacccgcagggcagagggggcagtttagatggagggctgtctgtcagccccttccatccactaacccatcactgcctcccagggcaggaaaccagggcagggccagcctgcgcattagggcagagaggaggggcaggtctcacgcccacagcccctccccactgagtcttagcatgaggcagcaacagaagctctctctttctcccagctaagtccgaggccccggtgcccagaaagggcagccgggatagtgaggttatttcctgcccgcccaggggcgccgccgaaggatctccagaatctgtgctcttcggtgcagccagtcctggggagtggggcgtggcgttgaaggggtcggccggggcacgaagaagctgtatcggaggcgtgtgtcctgggggttgccagccactaggacttgcagtgtcaaaggctgggccagtggcccatggcctgacagtgtctctgaggctgcagtggccccgctgtagcgcaagctgactgccccaggcagtaccacatctgtgggggagggcatcagcgtgtattcaccattgagggcataggagccatctggcagcttcagggccaagtagatgctccggtggccagggtttccctgctgccggacaagaatgtgggtggcccccgcggggatagtgaccacattgttgtatccgtacctgaatttcctgaaggagcctgactgcttgctgcaaccagaaccgtcccctccgcacaccatgcacttgtcaaacttcttcttggagccaatgatgcgatcacagccagcatggatgcatcggccctggacacagaccgaggagctgtccggggaacagggggtcccatctaccacccgtggctccagcacatagtagtagcccagtgcctgggcctggcaggtgagtttgcactggtcctggggggccacgcctgtgtagcgaggaacccagtccatgggccctgggaagctcttgaagaggtcggtgcggtggttgtaggcagcacactgctcctcgcggaaggtcagggctgagccagttgggcagtcctcagtgttgcaggagcggaagcgggtacggcggccctcacagtacttgccaccattccgggggacaggcctcgtgcagtctcgggaggagaactggacaccacccccacaggtccgagagcagtcaccccatggtccccaaggaccccagccaccagcctgtggaatattgaagtcctggagctggtccatgtggaggcagcgaccacccatgcaggcctgtgcgggcccgcagggtgtgccatcggcccagggcgagtgtttggtctggcacatggcatggccattgaggtggccagagcaccagagggcagcacagggcggcggcagctgtggacaatggcgtgagtcgggcccgaaggtcagctggcactggcggtcagcatcatagtccttgccagggaaagtcacaggcagatgcaatggagcctctggtttgtctaagagacagtgcccatagccattgtccaggaagtcagtgatgaagcgggcactgcagggggaccagggctcctcaggatccacatgagccatcacaggggccatgacatggcgagaggtgctcaaaggcccattcaaactgatgcatggcttggagttgtcatggagcatgttgaagacatgacccagttcatgagcagcagtgaaggctgactggagcccatcatcctccacaatggcacagctccgagccgggtcacagacggtgcccacatcagccatacccagcgtgtcgcaagtggagactccacacaggtcctgacgggtaaacagaatggctgtgtcaaagtggtcagggtccgagtcctcaggggtgttgaggccccgctgccaggcacagaagctgcgcagggtctgggcagcactgggccccacttggggcccctcctcgcctgaccccaggatcactagccgagtcaccaccaagctgacaggattgcggatgcttgggtgcttgaaggccttggctgctgctgccatcactgttagcaggtagcgctttagccccgcaccgtggaatgcggccatcttgtcatctgccaccaccagtgtctccacaaatctactcagtgaagcaaagcgcttggctcttcggggtctggggctggggcttccaagaggagccttgacgttgcacatgggaccttgaccgctggcaggactcttccggcgtaggatgtgagccccaggtcccccagcagagttaggggtgcctccctccaggggctggaggtggagttcagccccccgatattgtaacacgcctaacagggctcccccatcccagtgcagagatgccaccgactccggatctccattgatggtgccagtcaggtaggtgccaggctctgctccacccagcagctcaggcgcctggcccaggtactgcactgtcagcccctcgacctgcacaccggagtcctgctccagctctagtagcagcgtctccccaaaggcctgcaagcggcacaacagcctggcaggggcgcccgagccaggcaggacgctgccgttgagcttctctggaaacacgatctcctcctcccgggggagggggctggccagccgggctgagggcaggagagaggccagcagtagcagaagcagccacaccagccaggagagcggcacaatggggagcaggaggcagggttgggctccccacagccagcgccctgccaagcccctcccgggatgcgagcctgtctgggacatggcactggtactgcagctgggagggactgaggccgtctagggcaccaagtcctccacaccctagctttggaaagctcctctctgtagcctgggggcttggactcctgccaaggtcagaggcaaagttttcagaagggctgaggaccgttaaaggaaatggagaaaacttagtccttgggcttgggagaggtgcccaggggtctggcttctccaaactctcctcctgagccctcctttcctggatctttgtctctccctgcctgtgtcttctgcagcttctctggcctctccctctgtaggactctgtctgggccgcttctgtgcctgccctgtctctgccttcttccgctgtgcctttgtctctgtctctttcctcctctgtctctctcgtgcatatgtgtctgtgggtctccctgtgggttctccc

SEQ ID NO: 11190 - RNA, 1874 nt, Homo sapiens
  source 1..1874: mol_type = other RNA
ctgaatagctgggactacaggtgccagccaccacgcctggctaattttttgtatttttagtagagacgggatttcactgtgttagccaggatggtctcaaactccagacctcgtgatccgcccacctcggcctcccaaagtgctgggattacaggcatgagccactgcgcccggccaaaaaacaactctttaaaaatgtaccttagagcaacatgcaaagcttccctgctcagcaatcccaggttggggccccctgtcttcctatcgtcctacccgtcacaaccaccactgcaggcttctgatgctctgttttcctcctctgtctcagttcagttgctctgagttagagaggagctctctgggactggagctgactgcgccctggcccatttcctcactaccatcctcaagctcagatgctgacaggaaaatactgcctatgcctgaaggggcatcccttagcaggcggcccagttccttctcataacatttggctgcttgcagcagatctccattctgcttatgaattaatccttgaagataccaataatttggtgcattttgtggaagcagattttcagatacattctgtggttggtctttgatctcttccttgtcagttgattttttgcttatggacaaaccctctaaaccatgttgcacagcagtgtcttcagacttcccattatatttctgaaggttgcagtagcgctgatgggattgttgcttttcagcatcagggacttccttattgaatggtgtctgataacattccgtctccaggaactcagcgagatcggagtatgcattcagaggattcagtcccttctcaagagctttattcgaatagtccatagcatattgctttagtgcttcaatcatctctttatttccactagcttcagattctcctgtattctgcatttgtcttacttttgccttgtagcagcacccaatctggtgatagaggtagccattgtttggtgtggattccaacacccgttgaaacagttcaatagctttgtctaggtcaccttttcttctgtaaaatttggctgcactgcggaggacatctgtttggcaaggagacttttccaaggcttcttcaacaaactgctctccttcagcttctttattcatcttctgcagtttcaggcccaagagaaccttgacgtattggttatcaggactcagctcaatggcctgcttcaaaacatcagtagagaactgtttctctgggtgattatccagatggtacatcgcaattgccagtccagaggagaattctgggttgttgggcttttcttccagagccttctcaaaacacaccttcgccctttcatttcttccacacttcagttgtgtccacccttcctcacagtcaagttcagaatactcaatactgtatggatttgaaaatttcttgcaggtttgtttcaccttatctacataaatctgagcatctgagagtctgcccaagtgatagtagacccaggcgtagtttccccaagtgactagacttctgatttctgcttggtcagcatgttcttgctggattaactcttcagcttgccgtaagcattccagggctgcctcgttgttaccatctaggtgttttatgtaggccaacaagttgtacattgtagctttgaactcagtgtttaaaaattcaatctggttacacactctatcttctagatcccttgagacactgtcttccttgaataagttccaggtgaaatggcatttcagctgtggaaggattttctccagggaattcttggtgacctcactcatgactgccctctgtgtctctgctgttccgaaaagctggtgaccaggctgatttgttcttcagaagtcttcctgtctgc

SEQ ID NO: 11191 - RNA, 1891 nt, Homo sapiens
  source 1..1891: mol_type = other RNA
ctgaatagctgggactacaggtgccagccaccacgcctggctaattttttgtatttttagtagagacgggatttcactgtgttagccaggatggtctcaaactccagacctcgtgatccgcccacctcggcctcccaaagtgctgggattacaggcatgagccactgcgcccggccaaaaaacaactctttaaaaatgtaccttagagcaacatgcaaagcttccctgctcagcaatcccaggttggggccccctgtcttcctatcgtcctacccgtcacaaccaccactgcaggcttctgatgctctgttttcctcctctgtctcagttcagttgctctgagttagagaggagctctctgggactggagctgactgcgccctggcccatttcctcactaccatcctcaagctcagatgctgacaggaaaatactgcctatgcctgaaggggcatcccttagcaggcggcccagttccttctcataacatttggctgcttgcagcagatctccattctgcttatgaattaatccttgaagataccaataatttggtgcattttgtggaagcagattttcagatacattctgtggttggtctttgatctcttccttgtcagttgattttttgcttatggacaaaccctctaaaccatgttgcacagcagtgtcttcagacttcccattatatttctgaaggttgcagtagcgctgatgggattgttgcttttcagcatcagggacttccttattgaatggtgtctgataacattccgtctccaggaactcagcgagatcggagtatgcattcagaggattcagtcccttctcaagagctttattcgaatagtccatagcatattgctttagtgcttcaatcatctctttatttccactagcttcagattctcctgtattctgcatttgtcttacttttgccttgtagcagcacccaatctggtgatagaggtagccattgtttggtgtggattccaacacccgttgaaacagttcaatagctttgtctaggtcaccttttcttctgtaaaatttggctgcactgcggaggacatctgtttggcaaggagacttttccaaggcttcttcaacaaactgctctccttcagcttctttattcatcttctgcagtttcaggcccaagagaaccttgacgtattggttatcaggactcagctcaatggcctgcttcaaaacatcagtagagaactgtttctctgggtgattatccagatggtacatcgcaattgccagtccagaggagaattctgggttgttgggcttttcttccagagccttctcaaaacacaccttcgccctttcatttcttccacacttcagttgtgtccacccttcctcacagtcaagttcagaatactcaatactgtatggatttgaaaatttcttgcaggtttgtttcaccttatctacataaatctgagcatctgagagtctgcccaagtgatagtagacccaggcgtagtttccccaagtgactagacttctgatttctgcttggtcagcatgttcttgctggattaactcttcagcttgccgtaagcattccagggctgcctcgttgttaccatctaggtgttttatgtaggccaacaagttgtacattgtagctttgaactcagtgtttaaaaattcaatctggttacacactctatcttctagatcccttgagacactgtcttccttgaataagttccaggtgaaatggcatttcagctgtggaaggattttctccagggaattcttggtgacctcactcatgatggctgtttccctgcagttctgaaaagctggggtcccggttgattttgtttttagcttactgattccaagcaaatgctgaagaggtttccac

SEQ ID NO: 11192 - RNA, 1992 nt, Homo sapiens
  source 1..1992: mol_type = other RNA
ctgaatagctgggactacaggtgccagccaccacgcctggctaattttttgtatttttagtagagacgggatttcactgtgttagccaggatggtctcaaactccagacctcgtgatccgcccacctcggcctcccaaagtgctgggattacaggcatgagccactgcgcccggccaaaaaacaactctttaaaaatgtaccttagagcaacatgcaaagcttccctgctcagcaatcccaggttggggccccctgtcttcctatcgtcctacccgtcacaaccaccactgcaggcttctgatgctctgttttcctcctctgtctcagttcagttgctctgagttagagaggagctctctgggactggagctgactgcgccctggcccatttcctcactaccatcctcaagctcagatgctgacaggaaaatactgcctatgcctgaaggggcatcccttagcaggcggcccagttccttctcataacatttggctgcttgcagcagatctccattctgcttatgaattaatccttgaagataccaataatttggtgcattttgtggaagcagattttcagatacattctgtggttggtctttgatctcttccttgtcagttgattttttgcttatggacaaaccctctaaaccatgttgcacagcagtgtcttcagacttcccattatatttctgaaggttgcagtagcgctgatgggattgttgcttttcagcatcagggacttccttattgaatggtgtctgataacattccgtctccaggaactcagcgagatcggagtatgcattcagaggattcagtcccttctcaagagctttattcgaatagtccatagcatattgctttagtgcttcaatcatctctttatttccactagcttcagattctcctgtattctgcatttgtcttacttttgccttgtagcagcacccaatctggtgatagaggtagccattgtttggtgtggattccaacacccgttgaaacagttcaatagctttgtctaggtcaccttttcttctgtaaaatttggctgcactgcggaggacatctgtttggcaaggagacttttccaaggcttcttcaacaaactgctctccttcagcttctttattcatcttctgcagtttcaggcccaagagaaccttgacgtattggttatcaggactcagctcaatggcctgcttcaaaacatcagtagagaactgtttctctgggtgattatccagatggtacatcgcaattgccagtccagaggagaattctgggttgttgggcttttcttccagagccttctcaaaacacaccttcgccctttcatttcttccacacttcagttgtgtccacccttcctcacagtcaagttcagaatactcaatactgtatggatttgaaaatttcttgcaggtttgtttcaccttatctacataaatctgagcatctgagagtctgcccaagtgatagtagacccaggcgtagtttccccaagtgactagacttctgatttctgcttggtcagcatgttcttgctggattaactcttcagcttgccgtaagcattccagggctgcctcgttgttaccatctaggtgttttatgtaggccaacaagttgtacattgtagctttgaactcagtgtttaaaaattcaatctggttacacactctatcttctagatcccttgagacactgtcttccttgaataagttccaggtgaaatggcatttcagctgtggaaggattttctccagggaattcttggtgacctcactgtagtcctcgccattcgggaggctgagacaggaggatcacttgagcccaggaggcaaaagttgtagtgagctgagatcacaccattacactccagccagggtgatagagtgggaccctcatgactgccctctgtgtctctgctgttccgaaaagctggtgaccaggctgatttgttcttcagaagtcttcctgtctgc

SEQ ID NO: 11193 - RNA, 2013 nt, Homo sapiens
  source 1..2013: mol_type = other RNA
ctgaatagctgggactacaggtgccagccaccacgcctggctaattttttgtatttttagtagagacgggatttcactgtgttagccaggatggtctcaaactccagacctcgtgatccgcccacctcggcctcccaaagtgctgggattacaggcatgagccactgcgcccggccaaaaaacaactctttaaaaatgtaccttagagcaacatgcaaagcttccctgctcagcaatcccaggttggggccccctgtcttcctatcgtcctacccgtcacaaccaccactgcaggcttctgatgctctgttttcctcctctgtctcagttcagttgctctgagttagagaggagctctctgggactggagctgactgcgccctggcccatttcctcactaccatcctcaagctcagatgctgacaggaaaatactgcctatgcctgaaggggcatcccttagcaggcggcccagttccttctcataacatttggctgcttgcagcagatctccattctgcttatgaattaatccttgaagataccaataatttggtgcattttgtggaagcagattttcagatacattctgtggttggtctttgatctcttccttgtcagttgattttttgcttatggacaaaccctctaaaccatgttgcacagcagtgtcttcagacttcccattatatttctgaaggttgcagtagcgctgatgggattgttgcttttcagcatcagggacttccttattgaatggtgtctgataacattccgtctccaggaactcagcgagatcggagtatgcattcagaggattcagtcccttctcaagagctttattcgaatagtccatagcatattgctttagtgcttcaatcatctctttatttccactagcttcagattctcctgtattctgcatttgtcttacttttgccttgtagcagcacccaatctggtgatagaggtagccattgtttggtgtggattccaacacccgttgaaacagttcaatagctttgtctaggtcaccttttcttctgtaaaatttggctgcactgcggaggacatctgtttggcaaggagacttttccaaggcttcttcaacaaactgctctccttcagcttctttattcatcttctgcagtttcaggcccaagagaaccttgacgtattggttatcaggactcagctcaatggcctgcttcaaaacatcagtagagaactgtttctctgggtgattatccagatggtacatcgcaattgccagtccagaggagaattctgggttgttgggcttttcttccagagccttctcaaaacacaccttcgccctttcatttcttccacacttcagttgtgtccacccttcctcacagtcaagttcagaatactcaatactgtatggatttgaaaatttcttgcaggtttgtttcaccttatctacataaatctgagcatctgagagtctgcccaagtgatagtagacccaggcgtagtttccccaagtgactagacttctgatttctgcttggtcagcatgttcttgctggattaactcttcagcttgccgtaagcattccagggctgcctcgttgttaccatctaggtgttttatgtaggccaacaagttgtacattgtagctttgaactcagtgtttaaaaattcaatctggttacacactctatcttctagatcccttgagacactgtcttccttgaataagttccaggtgaaatggcatttcagctgtggaaggattttctccagggaattcttggtgacctcactgtagtcctcgccattcgggaggctgagacaggaggatcacttgagcccaggaggcaaaagttgtagtgagctgagatcacaccattacactccagccagggtgatagagtgggaccctgcctcatgatggctgtttccctgcagttctgaaaagctggggtcccggttgattttgtttttagcttactgattccaagcaaatgctgaagaggtttccac

SEQ ID NO: 11194 - RNA, 3929 nt, Homo sapiens
  source 1..3929: mol_type = other RNA
ctgaatagctgggactacaggtgcccaccaccacacccggctaatttttgtatttttagtagagacagggtttcaccatattggccaggctagtctcaaactcctgacattgtgatccacctgcctcagcctcccaaagtgctgggattacaggcgtgagccactgcgcccagcccaaaagtgactttttgtaaaaaattattttctacactaaaagaagataaataatagtcatgcaatcagaaattctacagaagtcagcaagatgttagaataaactggacctctgttttaaaacatgtagttttagtatttcataatacttaaaatttggatgttttattcttagtaaaattaacattacttcataaaataaaagaataaatctacttacaaaaatgtaattcaaaagttagactgtcaaataaattcagagctcctttctcagttcagatttttttctgtaataaaaggtttgataaatgacacaattctaatatgaagatccttaactacattaagcttgcttttattaagatctttatttatattcctaagattttaaaatcagcaaactcacttgatatagaggaagcacctacagattttggaagattttccttagctatctgcaaattgactgattaaattatggtaaatgcaggaacactgttttttctgttcacaccagaccctgagaaggcactgagaaatttgataagaacaaagccaataggagtgttgccactattgttttatgttcagtaaacatcagaattttaaatacatacagtaaatttatactgcaccaagggcacctgaaacagacatgccaaaaccacacactgtaacatctgttctaaactacagaaatgctaaatatcctatttcaaatactctaatttgtaaattaatacctgtgatgtcacaatgacactttttcataacaatcaaggaaagtaccattttcttgccaattttatggactaatttccttaactaaccctacaattatataacatttacctgtctttttttttttcttttaccatgctatacacaattacgagatacagaactaggcttaatcacactataataagaaaactcacttttgaattgtgatgtttctgttaacggaaggacaatacgttactataatacttttagtgtaataacttttgtttgaattatgaaaaaatttgaatcatttccctctagaccatttcatttcaaacttatactttgtttagtctagccagttgaccaaaaagaaagaaaataaaaggaaaaagatactcggccagatgagatagagagagaatgctaacacaaggttcaatgtatgcagttctcggttgctctgttccatatgcccacacagtgtcatgacatattggtgtacccctaaacagaacgccagatcagtccattcttactaggctgaagaaaattctctatcagagcatcaatgagtttcttcagttcttcctccagtaaagcagtgtcactctggtcaggtgacgcacacatctctgcataatactttatctttggttctgttccacttgtccgaagggtagcaacacagccattttgaaaagtaaatgtaatcatttggctgtttttactcacaggcagcactgatttcttattaggctggctactgtcatatccagtggtaacgtcccgtacatgcaatatagcaaatgttccacaaaattttggatattcttttggagaatcaaaattacgaagcctttcaaatatacttttgatggtaggtggttcataacacaagaaataggaagtttttgaaatatgataaccatatttttcataaaccttaaccagttgctgtttcaatgttatattcatggtttccaggtaagatgccatctcagcaaccacaacagctgcactcaccccatctttatccaaaactgaagttccacagagaaaaccaatagactcttcaaatgcaaaaaggacttctttcccattttccaggaggtctattatcctacttccaatccatttaaaacctggtaatgtttcttcaaaatgaaatccttctttaagtgcaattgccttcagaattttagaagagactgtggtggctaacatataaacgttcttcacatcagcatttcttgatttatttttcttccagcaatcaaacatccaccatccaaacaaagctgccaactcattccctgtgaaaactttccaacaaccattctcctgaagttctgctgctgccagtctgtctgcatcaggatctgtggctagcactacccgggcattttctttctctgccagtctcaaggaaagttccagcacagattctccttcttcaggatttggacatttaacggtagaaaagtctggatcaggatctttttgttctggtactggaattggaggcttaaaaccaaacactttaaaagccaactgcacatagtcatgtccgaccccatgaaaagatgtgtgcacaaatttcaaggtggtcttcgagtttaactccctgtaaaaacagatctttttcagatcttccatgtatctcctgcaaatgtcctgcagagggtctctcttcagcgggctggtatccactaaattatcattccaggaaccattccagggttccacacattcttctatacattttagaatttctttatcatgaggagatgtgatctgagcaccagtttcccagtaaaccttgtatccattgtcttccttgcggttgtgagaggcagtaatcatcacacctgcaactgctttgagcttctgaactgcatatggtacaaaaggtgtaggaacatatcttgaaaaaaggtacacaggaacatctttggccagcaagactgcagcagtgagtttagcaagcctctggctgctgcagctgctagttacttgaccccgagtgtcatacccaaccacaaagcctctctgcttgaagtctgagaaacatctctcaaggtatttgtacatcccctgtgttgactgtattactgtaaggtcattaatatagcaaaaccctgcccccatggcagaacgaagtcctgcagtcccaaaagtcattcggcaacaaagacgatctcgcagctccttgttcatcccattccgtaacaggttttcaatctgctcttttgttttgggattctgtaaaaaacaggaatcatgttctactcttcttcctgggcaccatgccagcctcccttggagcttatcccagcggagccactgcccgatggccgtgtccagctgagggtccccggtgtggtagggggcgtggagcaggttggagttcagatccccctctgtgttttcagccatggcgaccagacaggcgtacgggccgggggccggcgaagacactgagttggggtggggggtggcttggggttcgctcaccagggtccaggcgtccccacctcactgaagggcatcggagaccaaccgcagggtgttcgtaacagctcctgccgcggcgtcagggaaccgggagagagggggtttatggccgcctgctccccagcggaccaggtccgggtctctgggcgaagtgactgaggcggtcgcgccgcgagagaacaacagtcccagatgtctgggtcctggctccgccgccgccgccgccgcccgccccgcctacggccccgccccgcgccttaggccccgccccttcccgcccttgctgatttaagtccccgaagttctagactggagcccgggagcgcgctccccacgcctccgaagtagtgggggtttacagcccgtccgggtggtgaggcaatagtgcacggttctttttattttttaatttgccaagggtctcctttcctcgatctgctctcacggctaccactagcaagctgcctttgcgcttgccctgcaggtccccagcgcgcgcgcaggcccccagt

SEQ ID NO: 11195 - RNA, 3548 nt, Homo sapiens
  source 1..3548: mol_type = other RNA
ctgaatagctgggactacaggtgcccaccaccacacccggctaatttttgtatttttagtagagacagggtttcaccatattggccaggctagtctcaaactcctgacattgtgatccacctgcctcagcctcccaaagtgctgggattacaggcgtgagccactgcgcccagcccaaaagtgactttttgtaaaaaattattttctacactaaaagaagataaataatagtcatgcaatcagaaattctacagaagtcagcaagatgttagaataaactggacctctgttttaaaacatgtagttttagtatttcataatacttaaaatttggatgttttattcttagtaaaattaacattacttcataaaataaaagaataaatctacttacaaaaatgtaattcaaaagttagactgtcaaataaattcagagctcctttctcagttcagatttttttctgtaataaaaggtttgataaatgacacaattctaatatgaagatccttaactacattaagcttgcttttattaagatctttatttatattcctaagattttaaaatcagcaaactcacttgatatagaggaagcacctacagattttggaagattttccttagctatctgcaaattgactgattaaattatggtaaatgcaggaacactgttttttctgttcacaccagaccctgagaaggcactgagaaatttgataagaacaaagccaataggagtgttgccactattgttttatgttcagtaaacatcagaattttaaatacatacagtaaatttatactgcaccaagggcacctgaaacagacatgccaaaaccacacactgtaacatctgttctaaactacagaaatgctaaatatcctatttcaaatactctaatttgtaaattaatacctgtgatgtcacaatgacactttttcataacaatcaaggaaagtaccattttcttgccaattttatggactaatttccttaactaaccctacaattatataacatttacctgtctttttttttttcttttaccatgctatacacaattacgagatacagaactaggcttaatcacactataataagaaaactcacttttgaattgtgatgtttctgttaacggaaggacaatacgttactataatacttttagtgtaataacttttgtttgaattatgaaaaaatttgaatcatttccctctagaccatttcatttcaaacttatactttgtttagtctagccagttgaccaaaaagaaagaaaataaaaggaaaaagatactcggccagatgagatagagagagaatgctaacacaaggttcaatgtatgcagttctcggttgctctgttccatatgcccacacagtgtcatgacatattggtgtacccctaaacagaacgccagatcagtccattcttactaggctgaagaaaattctctatcagagcatcaatgagtttcttcagttcttcctccagtaaagcagtgtcactctggtcaggtgacgcacacatctctgcataatactttatctttggttctgttccacttgtccgaagggtagcaacacagccattttgaaaagtaaatgtaatcatttggctgtttttactcacaggcagcactgatttcttattaggctggctactgtcatatccagtggtaacgtcccgtacatgcaatatagcaaatgttccacaaaattttggatattcttttggagaatcaaaattacgaagcctttcaaatatacttttgatggtaggtggttcataacacaagaaataggaagtttttgaaatatgataaccatatttttcataaaccttaaccagttgctgtttcaatgttatattcatggtttccaggtaagatgccatctcagcaaccacaacagctgcactcaccccatctttatccaaaactgaagttccacagagaaaaccaatagactcttcaaatgcaaaaaggacttctttcccattttccaggaggtctattatcctacttccaatccatttaaaacctggtaatgtttcttcaaaatgaaatccttctttaagtgcaattgccttcagaattttagaagagactgtggtggctaacatataaacgttcttcacatcagcatttcttgatttatttttcttccagcaatcaaacatccaccatccaaacaaagctgccaactcattccctgtgaaaactttccaacaaccattctcctgaagttctgctgctgccagtctgtctgcatcaggatctgtggctagcactacccgggcattttctttctctgccagtctcaaggaaagttccagcacagattctccttcttcaggatttggacatttaacggtagaaaagtctggatcaggatctttttgttctggtactggaattggaggcttaaaaccaaacactttaaaagccaactgcacatagtcatgtccgaccccatgaaaagatgtgtgcacaaatttcaaggtggtcttcgagtttaactccctgtaaaaacagatctttttcagatcttccatgtatctcctgcaaatgtcctgcagagggtctctcttcagcgggctggtatccactaaattatcattccaggaaccattccagggttccacacattcttctatacattttagaatttctttatcatgaggagatgtgatctgagcaccagtttcccagtaaaccttgtatccattgtcttccttgcggttgtgagaggcagtaatcatcacacctgcaactgctttgagcttctgaactgcatatggtacaaaaggtgtaggaacatatcttgaaaaaaggtacacaggaacatctttggccagcaagactgcagcagtgagtttagcaagcctctggctgctgcagctgctagttacttgaccccgagtgtcatacccaaccacaaagcctctctgcttgaagtctgagaaacatctctcaaggtatttgtacatcccctgtgttgactgtattactgtaaggtcattaatatagcaaaaccctgcccccatggcagaacgaagtcctgcagtcccaaaagtcattcggcaacaaagacgatctcgcagctccttgttcatcccattccgtaacaggttttcaatctgctcttttgttttgggattcttatcccagcggagccactgcccgatggccgtgtccagctgagggtccccggtgtggtagggggcgtggagcaggttggagttcagatccccctctgtgttttcagccatggcgaccagacaggcgtacgggccgggggccggcgaagacactgagttggggtggggggtggcttggggttcgctcaccagggtccaggcgtccccacctcactgaagggcatcggagaccaaccgcagggtgttcgtaacagctcctgccgcggcgtcagggaaccgggagagagggggtttatggccgcctgctccccagcggaccaggtccgggtctctgggcgaagtgactgaggcggtcgcgccgcgagagaacaacagtcccagat

SEQ ID NO: 11196 - RNA, 7892 nt, Homo sapiens
  source 1..7892: mol_type = other RNA
ctgaatagctgggactacaggtgcccaccaccacacctggctagtttttgtaattttagtagagacggggtttcgccatgttggccaggattgtctcgaactcctgacctcaagtgacctatccgccacggcctcccaaagtgctgggattacaggcgtgaaccaccgtgcctggctgttaactagttttattaaaccctacaagctctaaaacacgagacaaggctttccagagtaaataggatgataaaaagttaaaattccctggaagagtctgttttcaccaacttgcaagaagtgaaagagccgatttctttctgtttattctttaaaaggtttggcctgcaccctcagtgcacactgtggaaggacagccccatagtcacaagggctgttcagggacagagcttcccatccatccaatccacagccaggaatcttgacggcagcaagagaaaagtcactcatcacctccgagagaggctccgtgagagacacagccaacttctcatcagaaaccatgagcatctgaacacgcggagtgcacattcagagcgcagaagagaaagggaactaggctgggcaagctgatggcagggctggtccagggacgggctgggactcccagccccaatctgttctcagggacgagaagtcctggctgagatccacgcagctcaggaaggtggtgaccccaggccatgggtcccgctgaggatgcctggaaatccgcatcaacccagctggctcaggtggagatggaggctccgggacagtgtgggatgggaggagggtgagtaaatgccaggcccggtccagggcctctccctggcctccagcctgcagcccaccctaacccttcctcagcagggctgatcactatcagggatggcccaggtgctgtcagagaagagggtgagccagctgtgtcctgtgtgcctgtgacaggtcccaatggcaggaacttcaggcagggaggcagagatcccacacagtcctgtcaccatggcagggcaggtgtgtgacccgggcgggttcacgtgcgcagcgtggagaggagtgtgcgctgggtgtaggacaatgggcgtggcaggtggggggaggcacaggtgggtgggtgtgacaggcacacaaccatcactgctgagcacctccctacaaagcgccagggggcccagggctaccagtcctgagggcccacaggggggctggcatccctggggaatccttgggccctatgccctcctggcagccctgtgacacatgccccaggtctgggatggtggcccagcaatgccctcagggccagggaagtgggtggaaggagaggagccgcgtccacactcctcctgagtttcctgagcactctccaggatcccaggccaccctggggtatccggccagggactaggaacctggcaagggcctgggcctgagataggtgagctccttccaccacctcaggcctcagggcccctcccacctctgagcccccacccaggctggctcccagagtcccccatcatccccatgaaatgtgtgcacatgcccctctcccaggtccccaccagcctctagggaacacgcctaccatgggggcggggtgggggcaaagcctccagagctgggctgggtggaggctgcaggtggccctgatgctcccccctctcccagacctgttcttgatccccaccccaaggttctcctgggccccacaggctgcgcctactcctaaccctgcagccagcaaagccctcacccctcccgagtgtggcaccggaagtccttgctggcctcctggccagatgagggctgccagaccggacgagacaggaccccgtgatggggaagggccttctctcggcctctgctcacgagctagagaccagcctcagggtggggctgggtgggagggatgagcacagctgcaccctacccaactcaccccaacccccagtcaccctctggcccacactgctccccacacctctgcccaggtctcataaatcctgcccagtggcccctccccacacagccccccaagagcagttccacttgggattgtcatggtacctgcagctcagcaagctgacatctgtgcttcccaccccaacaggggcagggagcccggatgaagaaagaatgagggcagagggcaccccatgcccaagacccacccaccccaggaccctccaagaggccatcagggcgacgccaacacacacacagacacacacacacacacacaaacaaacacacaattacaccccacagtgtggtcacttacaggaggtgagccttttccactggtgggtcaggcctcagtggggtcactgagaacccaccaaatcctcccaaatcccagcgtcagggctctgttggtctcgctccagttcaatccctctctccctctctctctgcagcttatcctgtctccgtatctttccccctcattctcggagtcactcagtctccctcttaaacaacaggtctctctcccactccacctcccaccatctctcccaatctctctcattcattttctgaaatattcaatccctttcacacacgactttctccgtctctctcattgatacacacactctccccccatccctgtctctctctcacacacacacacatgcacacacacacgcacacaggcagactcagccctccagggtctatgtctctgagctgagccccgctgagaggcaggcttgtctggggattgcagggagcactcacgcccacataggatgtgtccacgtggacagcgcttggccctttatgtacccactgtggatccttcactaggcaaccaggctggacttggaccagtgcaggtggaactaagccaagaccctgaaggccagggcagggtcagctccagcctcagcactcgccctaatccaggcacggtggagagtagcgtgagccaccaggcgggcccaagctgaagagctcaccgcatagcggggacagggatggcaggagacttgccactcagaccagggaaggatgacagggaccccaggcacaggcacaggtgtcagcagagaccacatcagtgggggtccccttgggcaggtggggggtggcatccagggctggagggtcacaggccactggcatggctcagcccagttctcacacagcatcctccatctctataatcatggggtcagtgtcacccctgggcatgaaatggagatactgctgttggcaaatgagcttggagagcagaggccaagacttctgggtgtcaagtgaggtgtcacaactggggcctgacttcatagaggccaaggtttcttcatagaggaagaaaccccgggagagtggctcccacggagggaactgccatgcacagctccgggggaggaggtggagcagtggccaccagccctgacagaaggcaatgcggggcccaggggcccagaaagaaagggcagagtgtggcctggtgaggccactgccccaagggcctatgcagtcccttgactgcgacctttgacaaagtgtgttacttgggtggggttggggggactccaagctgtgatgactcaggccagctggcaggagcgtgcatggtgaccgggatggagcagggttcagtgaagcaaccccatggatataagcacagggcccaccatggcacatgcaaaggaaggggaggagaaggaccgggttggcaacaaggagaaacccggctcaaagcaggtttgagggaggaagcagagaggacagttcagaggacagctttgcaactgaccagttagaaggcaaaggagcccaggccaggcacggtggctcaagcctgtaatcccaacactctgggaggccaaggtgggctcgcttgaggtcaggagtttgacaccaacctggccaacatgctgaaaccccctctcaactaaaaatacaaaaagtaaggccaggcacagtggctcacgcctgtaatcccagaactttggaaggtcaaggcggatggatcgcttgaggccaggagttccagaccagtctggccaacatggtgaaaccccgactctactaaaaatacaaaaattagccaggcctggtggcgcacacttgtaatcccagcacttggaaggctgaggcagaatgcttgaacgtgggaggcagaggttgcagtcagcccagatcacgccactgcactccagcctgggcgacagagctagactctgtctttaaaaaaaaaaaaaaaaaaaatagctgggcgtcatggggcacacctgtagtctcagctactggggaggctgaggcatgagaattacttgaaccctggaggcagaggttgcagtaggcccagattgtgccaacgcactccagcctgggcgacagaacgagaccctgtctcaaaaaaaaaaaaaaaaaaagccgggcacagtggtacacacctgtaatcccagcactttgggaggctgaggtgggtggatcgcccctgaggtcagcagttggagaccagcctgaccaacatggtgaaaccccatctctactaaaaatacaaaattagccgggcgtggtggcgtgcgcctgtagtcccagctactcgggagactaaagcaggagaattgcttgaacccgggaggcggaggctgcagtgagccaagattgtgccactgcactccagcctgggtgacacaatgacactccgtctcaaaaaaaaaaaaagaaaagaaaagaaaaagcagctcagctagcaggagagagccagcaccggagcctccacgcctggactttactctctggccccagtgggatcacctcctccaagaagtggcccctggtcctgctgaaggccccactctaagatgcagcgctctccacgctgtgtaagtccctggctaaggctccctgaccacccctgtacttgccggctcagcccaccaggtggcgcccgcgccatgcctcggccctgctggactccgaagccgccacttccctgcgggcgcctcctggtgtttgttcccttgggctcggcctggacagccctgctggttcccggagcctagcccagccccgcgagtgattcacagaactcacacctgacggtgggggaggaaggggagagcagcagccaagaggtgggtccaggctctcccaggggcgagtgacttcagtccagatgtcccctgaacccctggggattccgcatcaggaccagggcctcccatgtccagaccccacattcccgtcagtgtgtcccggggagcacggagggacctccacactgcatttcatggggcgaccgcccttaacacccggacacacacggaaccccacactaccctaaagtctgaaaggtggacacgcgtggcgaagttttagaggaatttcaggacaaaagtcctgaaaccacaaggttcttaccacctgaaaaccagctccgtaacagacaaactagacacttgtgagtttgccggcatttgctttaaaaataacaaggctggtccaagatcttagaagaaaattatattcttttaaagaaaatgaaaatatcctcaagggaaaaacttaatttaagtcaaatcttgtccttttgtcgtggagccccttgccccgcgcgcagacacaggctttcctgaagcgtggccagggcgcccctctcatcgctcctgagcgtgacccggggctggagccgcacggggattttcccgagctgagcaggggggtcggggggcccaagccaggagccctggaagagggagcagggcggcaactggggccgcaaacacccatcaaagtccccaggaccaattcccacagacaccacgtggccacaggcagtgccctttgcaggccccctccccaagggtgtcacccctcaccccctcctgggaccccgcctaaaccaggcacccttccacccaccagcaggaactgcgctaggagatgcaggaacacccatgtccccgccagccccgccttccagaccacaccctgcccgggagtgcgctttgcgaggtcggggtcgggggggagggcgggggccaggcccctgaacaacagacagcagctcccacccagcaatgcagccgggtcacctcgcacccctggccaaggcaggggccctctccagcctggtgacccacggcctaccctgaggctgcagggcacagggggcctccaagtggaaagctggtgatggggtgggtgggaggcagggcccgcagggaagtgacttgagcaggcacagacggtgaataaatagaagcttccacgcgggggtccggcccctgcagacagcagctcggtgggaaactgattggagggagctcccctgacgctgaccagggccacccacgcgggccctccctccacacccacacccaccccggcccagggacgggttttcccctgctcagagctcagtgacgtgcacagtgggtgagggaagaggcccaggttggaggcgccgcaggtggcaacgacgacacagtaggtggcccgccaggggatagcaacggcgtccctcctccccgctcagctgcagcccgcagtcctcacagtggtaacatgccacgtggtagtctctgtccatggacaccacacggatggttgtctcgcagccctgtgcagggaggataggacgggcacaggaggcgcattttggtgcaaaaaccgtgtgatagtctcgcacgcagtagatgttgttctccacgtccacggtgaagggaaccccgtccaggcactcattgcacacggagcaccggaagcagcctgggtggtaggacttgcccagggcctgcaggatcatttccatgatgagatgtccacacacgctgcatttgtcggccgtctgctggaacccggagtacaggaagtcctcctggcagtacactttctcacccacgttgtagaacgccttcccacggagtcgtctcccacacgagtcgcaggtgaagcagtcagtgtgataaagactccccattgcctggcacgcctgctgggctccgtagatgccaagcccacacttgatgcaaatgccgaagtagtcccgcgccgtgcgcgcctcgagcgcccgctccagctcccgggtgagcgcctccagccgccgctcggccgcgcttgggccgccctcccggccagggggcagcgggagtgcaggcagcgggaagggagccggccccgcaggctccggggagcgagcgggcgcggggcaggcgccgggcgggaggaagtcagcgtaggcgccggccgagccccgggagccgaggctggaaacgctggagcgggcgctgcccaccgaaggcggcccgggaccgggacgcgggtccgagcgaccggagcgcgggctgccgtggcgctggtcgtagcccaggctgatgccgctggatcgggcgctgccgccaccgccgccgccgtcggaccccgccaggctggcccgtgggctgcccgcaggctgcgcgctgagctccggaaccgccgcgcgccggggaccccgctccccgcggctcagtccgtccgccccggcctcggggccgccgctgcccttccctctgcggcccagcgcgggcgccgcctcgtctccaggcccaggccgcggcccccgccgcccccgaccgggagagccgcacccgggctccagctcccgcagggccagcccggccaggagtagggccgcctcgtccgcgcccgccctggagcgctgcatggcccggcccgccggccctggcgcgtcacctccgcctccgcttcccgccgccgctccggccgggccgccgcatcgtccgcccgaagcccggagcccgccccgggacccctgggcgcggggcggggcggggccggcgccgggccggggtcgttccggcggccacgcgcgggccgggggacgcggcgccctgctcggcggcgcgcgcggcggaggaatg

SEQ ID NO: 11197 - RNA, 2978 nt, Homo sapiens
  source 1..2978: mol_type = other RNA
ctgaatagctgggactacaggtgcccaccaccacatctggctaattcttgtatttttcatagagacaaggtttcactatattagccaggctggtcttgagttcctgaccttttgatccgcctaccttggcctcctaaactgctgggattacaggtgtgagccaccgcatctggcccaagtttttttctataaaaccacatattgcactcagggtagggtaaatgatgcatcatgcctgctggcaacatgggccctatctggaaagcgagtgcccaccaccatagcacagttccatgcagtgcctgtgtggtgctgaatctcaggagcagccccaatcctgtgaaccacaactacagggaccttagacataagcaaatacttctggtggccaggcctgccagcaagcagatgctaaccctgtcctgggggcctgcagagaggtcgggccagtgcagaggtggtgagacccatgtctggtctccccaactcccacccatgctatgcaatgggggcgaccacgcacccgatctgcctgggagggtcctagtgtgcccactgccttgctgagttatgagggatgctgcctctcacatctcaccggtatcgcatttgaaggacaaattatgtcttcccttccccaccctgtggacctccgtttcctcatgtgcaagtgggggatgataggcttacatggttatgcagtgggggtatcaatgggatccatctgtcaataccttgcatccagtgaccacctggagcacacctgcagttcgcaagttaggcttcctgctgcagtgaggggagcaagcactgcctggagccagggagcttctctgaaggaggtgttggaaaggacttgttccagaatttgggcttgtattgggagcttgggggaaggttgaaagaagcctttgctccagattggatgctgtcagaggcagggtggattctatcacctggcatcttccccaatcttacctgaattttccatttgagagcattttcagcttctggaaacagacatttcacccaaaattccagattccctgcttctctggctaattctttgtatatttgaagagacagggtttcactgtgttggccaggatggtcttgatctcctgacttcgtgatccgctggcctcagcctcccaaagaactgggatgagaggtgtgagccactgcacccggcctcaatgtagcttattatcaaagtatttacacagaaaaattaatcaaagggcacaagcatttcaatacttaggttaagatgaaatctgtggccggaagagggccagacacacatgaaatgttttgtgcatgaaggaaccacaacttaaaatgattttctgttattcgttttggtatgttattttggaaatgtgattaatcacgtatgtaaaggacgttgggaagaatttccagatactctgatatgcatgacatcttaatcacacaatataaagcaaggctatcttaggaaattaggtatcactgccaaggacctttacatgagatgataaattaaaattactattaaatttgtaacagtcagatgggctggcaggcaagttgcgtcatttttttctcagtattttttctttttccttgattcaataaaacaaacttaaatgccagttatctgcagaaccctcactagactatgtttaatgatatgtgaaacacagcctgcacactcacagatccttgccacgtcccgttcccatcctctcaaaacctgtgttaccctgtggctagatttctcaaggagatgaaagagagagacgaatgagaaccaccttctttcaggtcgctctgcactgctcctgcaggtagacaatgacctctccggtgaggctattatccttggcttgggggtggaggcctttatcctggaaaagaggcctctcagggtggggaggtgatttaaattcttatgagagagacgcagctccccatctcatctggaccttcacaaacctaaactggaaccgccagaaaaatgactgacaacgggccacgcaagccaggcagagacgcggggagaggctgaccacaagaaaggcggacgtagaagataccgtcctctggcgcacagggcacatatgtcccaacacacacacacacacacgcacacagggacacagagcaaaagagtgagaaaagggagagagagaaacaagagagagacatacgcacacacacaaacgcacagacatacagcagtggcacggtaacacctacacccaggcagcccctgaattttcagggttctgctctccacgactacaacccactagtgagagagcagcccacgggcacacaagcaaacctctccttttttgaagagactcactggcacaccgtccgtgcaggcctgaacctgggatcccgcgctgcttgcccggccctccacctgcagtttcttcctcctggacgaccctccgtgaatcccggcctccagagactatcctgttgatgccctggccaggactggtcttagccccgacactgactaatccctctagtaccaggtactcgggaggcggaggcaagagaatcacttgaacctgggcggcagagtttgcagtcagctgagatcccgccactgcactcgactgagtgacagagtgagattccgactattaaaaaaaaaaagatagaaaagaaaaatgaccgcggagcggcggctgcggggactggggcggcggcgggtgaagtgaagattgggaaaagggcttcgtcgacccttcccgaatccgggcctgaggctgggatctcgcgctgccgcccggcgatccgcctgaggtttctaccttctgaggtttcttcctggtggtcagccctccgagaatcccaggctccggagaccatcctgttaaagccctggccaggactgctctcaggcccgactctgacgcactatcacacagggctcctacttcgcaaagtctcagggacccatccacggcaacagt

SEQ ID NO: 11198 - RNA, 2868 nt, Homo sapiens
  source 1..2868: mol_type = other RNA
ctgaatagctgggactacaggtgcccaccaccacgcccagcccattttttttttttttttttttttagtagagatggggtttcactgtgttagccaggatggtctcgatctcctgacctcgtgatccgccctcctcggcctcccaaagtgctgggattacaggtgtgagccaccgcgcctggccaaccctgctcttgaaatgtctaaatcttttcctcactagcatatacaattcaaatgcacaggcctccatgacttctttggaatttaaaagaagccttcatttcaaggatagaaatatgtaaaattttaccaaccatggataagtttgttatgggagtagtggaaggacagtggaaaaaaaaataggttttttcatgatacttttatttttccttttttaaaaataaatttagggggtacaagtacagtttagatacatgaatatattgtgtagtcgtaaagtctgggcttctagtgtaaccatcacgcaaatatacttgtatttttctaattacagttctaccaaacatttgccaccacaaaatacaagtatttttattctttatttaaattatggtgagtgatatttcttcctatatagccattaagatctctggaagttttgatctactttattcaaaccactttaataaataagacttttcacctaaatgaaatacctttgaattttataaacaacttccatgaaacatatattaaaaccacctttaatttggtatgaagacactttggcaatgcagcggaataaatgatcttggcaagacccagcaagtacagtaaatgctcatgagctctatgaaaaatataggctacagaatacttcatttttcttttattgaactacagtacaaatgtgactgcttcaatatgaacatctatcttccaccaaatagcaaacaggcatcttatgtaattaaaaactaattatttcaattccaccaatggaaaagcaaaacaagttgcaaatatcaacaatacagagcctgctggtaaagatagagatgagtaagttataagctaataaagctgcagcctgaggatgccagatcaacattataaatatgaagaaaaagaaactaaatatttactcatcgcaaataactcggcataagcaccagctatgttcaggtgcggccagcacataggccaagtataaatgtacaatcacagtgaactaaagccataaaatctagttccctgacccttcaatcaaccattcagagcaatgggaatatagcggggagacagaagtcccactttggttgctcatattacattaagccagcctgccccaccccaatccccttcccaccaataaaaaagtcaccgtgagtgtataattggtcaatccagtttatccaaggtctatagatatagccatgatttgtcctatattcatgttaaatagaatgcttacataaaattaatactcaaagacattgagctgatgtgcatgtatattcttatttaacatttaagtggctttaatggtattttagaatgtcacctatggcatgagtcttcaaatctggattgaagactgtggcggttttataactgcatgtaagatcttaaatgtaagactctgggcctacctacattaaggcaggtgacagtaccctcattcattctacataataaatacactcttctgtgactgcaaaattctgaatccttgaatgatttactataataggctaaggttgtataaggcacttttggctctgaaatatttctcctaactctcaggctgaatcttaaagaaatatttacaaagctgcaacaaattaattttagaaccggatgctttattcgtaggtctaatggggatggtgagaagcaatttgtacacaatgcccattaatctctcactgtgccatgtatcaatcatagagaagatcccaggcatgggccacctgaactactatgtcgcttacttgacttctcaacagccacatgcccctttctccttttcttcacttaactgatccgtagaggcatgaccatttgatcgcaccactccttcaggaatccaggacttgtccacacaccgttccattcgcttcattatcaggtccagaagcatctcaattgcttggcttatgtttgtcccattggcagcactagtttcaaagtaggggattccatatttctctgcgagtgctatggcttcctcctctttcactactctctggtcctccagatcactcttgtttccacacagcactatatctgggttttcacaatatgcatgcatctgtagctggcttatccagtttctgacattgaggaaactttgctcatttgtcagatcaaaaagtagaagaaaacccatagcatctctgaagaacgctgtcgttaagctacgaaacctctcctgccctgctgtgtcccataactgcaggtggattctctggcctctgccagtggctccatccggcccactggctctgtacaccactcttttttccctgaaatcaatgcccactgttgtgataaatttggagttaaatttaccatctgtatattggtaaagtacactggtcttccctacaccagagtctcccaaagctaaaaacttgatgaggtaatcataatctccatcagacataatgaagaactcagtagttcaccaagtcaagcagagctgggtttgaatcccaaatctcccagataccaattacttggatgtctttgagccttagatttccaggtttctgttctttacagggtagagaaccgcttgttatgattttctaaaacgttagagactggagttaccaatgcttcaacaattgacaacttccaatcacatgtcctcttcaggaaggttactttttgtct

SEQ ID NO: 11199 - RNA, 2964 nt, Homo sapiens
  source 1..2964: mol_type = other RNA
ctgaatagctgggactacaggtgcccaccaccacgcccagcccattttttttttttttttttttttagtagagatggggtttcactgtgttagccaggatggtctcgatctcctgacctcgtgatccgccctcctcggcctcccaaagtgctgggattacaggtgtgagccaccgcgcctggccaaccctgctcttgaaatgtctaaatcttttcctcactagcatatacaattcaaatgcacaggcctccatgacttctttggaatttaaaagaagccttcatttcaaggatagaaatatgtaaaattttaccaaccatggataagtttgttatgggagtagtggaaggacagtggaaaaaaaaataggttttttcatgatacttttatttttccttttttaaaaataaatttagggggtacaagtacagtttagatacatgaatatattgtgtagtcgtaaagtctgggcttctagtgtaaccatcacgcaaatatacttgtatttttctaattacagttctaccaaacatttgccaccacaaaatacaagtatttttattctttatttaaattatggtgagtgatatttcttcctatatagccattaagatctctggaagttttgatctactttattcaaaccactttaataaataagacttttcacctaaatgaaatacctttgaattttataaacaacttccatgaaacatatattaaaaccacctttaatttggtatgaagacactttggcaatgcagcggaataaatgatcttggcaagacccagcaagtacagtaaatgctcatgagctctatgaaaaatataggctacagaatacttcatttttcttttattgaactacagtacaaatgtgactgcttcaatatgaacatctatcttccaccaaatagcaaacaggcatcttatgtaattaaaaactaattatttcaattccaccaatggaaaagcaaaacaagttgcaaatatcaacaatacagagcctgctggtaaagatagagatgagtaagttataagctaataaagctgcagcctgaggatgccagatcaacattataaatatgaagaaaaagaaactaaatatttactcatcgcaaataactcggcataagcaccagctatgttcaggtgcggccagcacataggccaagtataaatgtacaatcacagtgaactaaagccataaaatctagttccctgacccttcaatcaaccattcagagcaatgggaatatagcggggagacagaagtcccactttggttgctcatattacattaagccagcctgccccaccccaatccccttcccaccaataaaaaagtcaccgtgagtgtataattggtcaatccagtttatccaaggtctatagatatagccatgatttgtcctatattcatgttaaatagaatgcttacataaaattaatactcaaagacattgagctgatgtgcatgtatattcttatttaacatttaagtggctttaatggtattttagaatgtcacctatggcatgagtcttcaaatctggattgaagactgtggcggttttataactgcatgtaagatcttaaatgtaagactctgggcctacctacattaaggcaggtgacagtaccctcattcattctacataataaatacactcttctgtgactgcaaaattctgaatccttgaatgatttactataataggctaaggttgtataaggcacttttggctctgaaatatttctcctaactctcaggctgaatcttaaagaaatatttacaaagctgcaacaaattaattttagaaccggatgctttattcgtaggtctaatggggatggtgagaagcaatttgtacacaatgcccattaatctctcactgtgccatgtatcaatcatagagaagatcccaggcatgggccacctgaactactatgtcgcttacttgacttctcaacagccacatgcccctttctccttttcttcacttaactgatccgtagaggcatgaccatttgatcgcaccactccttcaggaatccaggacttgtccacacaccgttccattcgcttcattatcaggtccagaagcatctcaattgcttggcttatgtttgtcccattggcagcactagtttcaaagtaggggattccatatttctctgcgagtgctatggcttcctcctctttcactactctctggtcctccagatcactcttgtttccacacagcactatatctgggttttcacaatatgcatgcatctgtagctggcttatccagtttctgacattgaggaaactttgctcatttgtcagatcaaaaagtagaagaaaacccatagcatctctgaagaacgctgtcgttaagctacgaaacctctcctgccctgctgtgtcccataactgcaggtggattctctggcctctgccagtggctccatccggcccactggctctgtacaccactcttttttccctgaaatcaatgcccactgttgtgataaatttggagttaaatttaccatctgtatattggtaaagtacactggtcttccctacaccagagtctcccaaagctaaaaacttgatgaggtaatcataatctccatcagacataatgaagaactcagtagttcaccaagtcaagcagagctgggtttgaatcccaaatctcccagataccaattacttggatgtctttgagccttagatttccaggtttctgttctttacagggtagagaaccgcttgttatgattttctaaaacgttagagactggagttaccaatgcttcaacaattgacaacttccaatcacatgtcctcttcaggaaggttactttttgtctggctcgccccgccgtcctgtccccgcctggctcgggtcctcgcgcgccgcgtccacccgccgccggccttttttgggtcgttggcgggtattttcc

SEQ ID NO: 11200 - RNA, 2760 nt, Homo sapiens
  source 1..2760: mol_type = other RNA
ctgaatagctgggactacaggtgcccaccaccacgcccagcccattttttttttttttttttttttagtagagatggggtttcactgtgttagccaggatggtctcgatctcctgacctcgtgatccgccctcctcggcctcccaaagtgctgggattacaggtgtgagccaccgcgcctggccaaccctgctcttgaaatgtctaaatcttttcctcactagcatatacaattcaaatgcacaggcctccatgacttctttggaatttaaaagaagccttcatttcaaggatagaaatatgtaaaattttaccaaccatggataagtttgttatgggagtagtggaaggacagtggaaaaaaaaataggttttttcatgatacttttatttttccttttttaaaaataaatttagggggtacaagtacagtttagatacatgaatatattgtgtagtcgtaaagtctgggcttctagtgtaaccatcacgcaaatatacttgtatttttctaattacagttctaccaaacatttgccaccacaaaatacaagtatttttattctttatttaaattatggtgagtgatatttcttcctatatagccattaagatctctggaagttttgatctactttattcaaaccactttaataaataagacttttcacctaaatgaaatacctttgaattttataaacaacttccatgaaacatatattaaaaccacctttaatttggtatgaagacactttggcaatgcagcggaataaatgatcttggcaagacccagcaagtacagtaaatgctcatgagctctatgaaaaatataggctacagaatacttcatttttcttttattgaactacagtacaaatgtgactgcttcaatatgaacatctatcttccaccaaatagcaaacaggcatcttatgtaattaaaaactaattatttcaattccaccaatggaaaagcaaaacaagttgcaaatatcaacaatacagagcctgctggtaaagatagagatgagtaagttataagctaataaagctgcagcctgaggatgccagatcaacattataaatatgaagaaaaagaaactaaatatttactcatcgcaaataactcggcataagcaccagctatgttcaggtgcggccagcacataggccaagtataaatgtacaatcacagtgaactaaagccataaaatctagttccctgacccttcaatcaaccattcagagcaatgggaatatagcggggagacagaagtcccactttggttgctcatattacattaagccagcctgccccaccccaatccccttcccaccaataaaaaagtcaccgtgagtgtataattggtcaatccagtttatccaaggtctatagatatagccatgatttgtcctatattcatgttaaatagaatgcttacataaaattaatactcaaagacattgagctgatgtgcatgtatattcttatttaacatttaagtggctttaatggtattttagaatgtcacctatggcatgagtcttcaaatctggattgaagactgtggcggttttataactgcatgtaagatcttaaatgtaagactctgggcctacctacattaaggcaggtgacagtaccctcattcattctacataataaatacactcttctgtgactgcaaaattctgaatccttgaatgatttactataataggctaaggttgtataaggcacttttggctctgaaatatttctcctaactctcaggctgaatcttaaagaaatatttacaaagctgcaacaaattaattttagaaccggatgctttattcgtaggtctaatggggatggtgagaagcaatttgtacacaatgcccattaatctctcactgtgccatgtatcaatcatagagaagatcccaggcatgggccacctgaactactatgtcgcttacttgacttctcaacagccacatgcccctttctccttttcttcacttaactgatccgtagaggcatgaccatttgatcgcaccactccttcaggaatccaggacttgtccacacaccgttccattcgcttcattatcaggtccagaagcatctcaattgcttggcttatgtttgtcccattggcagcactagtttcaaagtaggggattccatatttctctgcgagtgctatggcttcctcctctttcactactctctggtcctccagatcactcttgtttccacacagcactatatctgggttttcacaatatgcatgcatctgtagctggcttatccagtttctgacattgaggaaactttgctcatttgtcagatcaaaaagtagaagaaaacccatagcatctctgaagaacgctgtcgttaagctacgaaacctctcctgccctgctgtgtcccataactgcaggtggattctctggcctctgccagtggctccatccggcccactggctctgtacaccactcttttttccctgaaatcaatgcccactgttgtgataaatttggagttaaatttaccatctgtatattggtaaagtacactggtcttccctacaccagagtctcccaaagctaaaaacttgatgaggtaatcataatctccatcagacataatgaagaactcagtagttcacctaatggacaaggtcaaatcagatatatttcttattgcttctcaaagtctttccttatttcacctattattcagtatgcagagtctcagaactgactgtttgc

SEQ ID NO: 11201 - RNA, 4280 nt, Homo sapiens
  source 1..4280: mol_type = other RNA
ctgaatagctgggactacaggtgcccaccaccacgcccagcccattttttttttttttttttttttagtagagatggggtttcactgtgttagccaggatggtctcgatctcctgacctcgtgatccgccctcctcggcctcccaaagtgctgggattacaggtgtgagccaccgcgcctggccaaccctgctcttgaaatgtctaaatcttttcctcactagcatatacaattcaaatgcacaggcctccatgacttctttggaatttaaaagaagccttcatttcaaggatagaaatatgtaaaattttaccaaccatggataagtttgttatgggagtagtggaaggacagtggaaaaaaaaataggttttttcatgatacttttatttttccttttttaaaaataaatttagggggtacaagtacagtttagatacatgaatatattgtgtagtcgtaaagtctgggcttctagtgtaaccatcacgcaaatatacttgtatttttctaattacagttctaccaaacatttgccaccacaaaatacaagtatttttattctttatttaaattatggtgagtgatatttcttcctatatagccattaagatctctggaagttttgatctactttattcaaaccactttaataaataagacttttcacctaaatgaaatacctttgaattttataaacaacttccatgaaacatatattaaaaccacctttaatttggtatgaagacactttggcaatgcagcggaataaatgatcttggcaagacccagcaagtacagtaaatgctcatgagctctatgaaaaatataggctacagaatacttcatttttcttttattgaactacagtacaaatgtgactgcttcaatatgaacatctatcttccaccaaatagcaaacaggcatcttatgtaattaaaaactaattatttcaattccaccaatggaaaagcaaaacaagttgcaaatatcaacaatacagagcctgctggtaaagatagagatgagtaagttataagctaataaagctgcagcctgaggatgccagatcaacattataaatatgaagaaaaagaaactaaatatttactcatcgcaaataactcggcataagcaccagctatgttcaggtgcggccagcacataggccaagtataaatgtacaatcacagtgaactaaagccataaaatctagttccctgacccttcaatcaaccattcagagcaatgggaatatagcggggagacagaagtcccactttggttgctcatattacattaagccagcctgccccaccccaatccccttcccaccaataaaaaagtcaccgtgagtgtataattggtcaatccagtttatccaaggtctatagatatagccatgatttgtcctatattcatgttaaatagaatgcttacataaaattaatactcaaagacattgagctgatgtgcatgtatattcttatttaacatttaagtggctttaatggtattttagaatgtcacctatggcatgagtcttcaaatctggattgaagactgtggcggttttataactgcatgtaagatcttaaatgtaagactctgggcctacctacattaaggcaggtgacagtaccctcattcattctacataataaatacactcttctgtgactgcaaaattctgaatccttgaatgatttactataataggctaaggttgtataaggcacttttggctctgaaatatttctcctaactctcaggctgaatcttaaagaaatatttacaaagctgcaacaaattaattttagaaccggatgctttattcgtaggtctaatggggatggtgagaagcaatttgtacacaatgcccattaatctctcactgtgccatgtatcaatcatagagaagatcccaggcatgggccacctgaactactatgtcgcttacttgacttctcaacagccacatgcccctttctccttttcttcacttaactgatccgtagaggcatgaccatttgatcgcaccactccttcaggaatccaggacttgtccacacaccgttccattcgcttcattatcaggtccagaagcatctcaattgcttggcttatgtttgtcccattggcagcactagtttcaaagtaggggattccatatttctctgcgagtgctatggcttcctcctctttcactactctctggtcctccagatcactcttgtttccacacagcactatatctgggttttcacaatatgcatgcatctgtagctggcttatccagtttctgacattgaggaaactttgctcatttgtcagatcaaaaagtagaagaaaacccatagcatctctgaagaacgctgtcgttaagctacgaaacctctcctgccctgctgtgtcccataactgcaggtggattctctggcctctgccagtggctccatccggcccactggctctgtacaccactcttttttccctgaaatcaatgcccactgttgtgataaatttggagttaaatttaccatctgtatattggtaaagtacactggtcttccctacaccagagtctcccaaagctaaaaacttgatgaggtaatcataatctccatcagacataatgaagaactcagtagttcacctggctcgccccgccgtcctgtccccgcctggctcgggtcctcgcgcgccgcgtccacccgccgccggccttttttgggtcgttggcgggtattttccgcctggccccacatcacttcccgtaaaggagagcgaggtggggcgggaccttctctcctccacctcccgccttctcctgtcacctcgggagcggcccccgcccggctggcggggggcggggtgctgtcgcgctctccccggcggccgcgcctccgaggggtcctctgtgagccccgaaaaggccccgctcgcctcctttgtcccaacactagtttccgctgccccattctggaaggcgctacaaaatataggagtgttttcgttttgggacacaggagggacatttacaaactgcaccaaggaccggtgcgcggcgaggtgtcgtttggggactctcccctattcacctccccaaaaagccatgttctaagggtgttttccacggcatcagttcgcggtcgccaccgtagcagccggaggtgccgggcgtactcacgccggccccgcccgaggttcccgagtccgcgcggctcctgaggcggcgtcccaggcccggccctgcccccggcttcccgcccctgcggctcctggcttaggtcggcctggacacggcgtttccggggcaagggaatgcccaggattcctggaaataacatgggagaaaaataagtaaaaaatttcgcaggaaaaaaatcaatgtaattccgggaggaaatggcaaacggagtctctgctcacactgtgtaattcaagaatataaaaccactgtaaatttctaagagtgttagagcaatgagtttaaaaagaagaaaactacagtatgttaaggaaccgcctctgtcggaagaaacctgcgcgcctttgctgccacccagcggctctcttctcccagcgccaacggtgtcgctccggcctgcggggtagtgaacctgggactgcgtagggggtcagacctcgtggttcccactcagaggcagccaagttcatccctctcagtggccaggaggtgtgaacagcagcccttgggcctgtccctatggagtctaaggcaaaggccctttgaaccaaatgtttccacttctaagcagagtaaaatgttgagaagccttagttcagcttcccttctgccttctaagccgtctcgctgacttgtgtctacctccaccgcaaattccagctgtcgcaggcccacccggtcaactccatcacctttccagtctgtagctactcacagttggcattacagcagttagcttctcaggtgggtccaatttacaaaatcacatataggatgaaccatatgaaattacaaacagttggcaatttcatacatttgatataacatttccaggcaaacataacacagtaaactcgggtttagagataacaaatgtcctaacaggttgataacttcaagagctcttcccgtgtgagagaagggccatcagactgttggtgaggttaagagagaaaaaggccgggttaggtggctcacgcctgtaatcccagcactttgggagcccgaggccggcagatcacgaagtcaggagatcgagaccatcctggctaacacggtgaaaccccg

SEQ ID NO: 11202 - RNA, 2956 nt, Homo sapiens
  source 1..2956: mol_type = other RNA
ctgaatagctgggactacaggtgcccaccaccacgcccagcccattttttttttttttttttttttagtagagatggggtttcactgtgttagccaggatggtctcgatctcctgacctcgtgatccgccctcctcggcctcccaaagtgctgggattacaggtgtgagccaccgcgcctggccaaccctgctcttgaaatgtctaaatcttttcctcactagcatatacaattcaaatgcacaggcctccatgacttctttggaatttaaaagaagccttcatttcaaggatagaaatatgtaaaattttaccaaccatggataagtttgttatgggagtagtggaaggacagtggaaaaaaaaataggttttttcatgatacttttatttttccttttttaaaaataaatttagggggtacaagtacagtttagatacatgaatatattgtgtagtcgtaaagtctgggcttctagtgtaaccatcacgcaaatatacttgtatttttctaattacagttctaccaaacatttgccaccacaaaatacaagtatttttattctttatttaaattatggtgagtgatatttcttcctatatagccattaagatctctggaagttttgatctactttattcaaaccactttaataaataagacttttcacctaaatgaaatacctttgaattttataaacaacttccatgaaacatatattaaaaccacctttaatttggtatgaagacactttggcaatgcagcggaataaatgatcttggcaagacccagcaagtacagtaaatgctcatgagctctatgaaaaatataggctacagaatacttcatttttcttttattgaactacagtacaaatgtgactgcttcaatatgaacatctatcttccaccaaatagcaaacaggcatcttatgtaattaaaaactaattatttcaattccaccaatggaaaagcaaaacaagttgcaaatatcaacaatacagagcctgctggtaaagatagagatgagtaagttataagctaataaagctgcagcctgaggatgccagatcaacattataaatatgaagaaaaagaaactaaatatttactcatcgcaaataactcggcataagcaccagctatgttcaggtgcggccagcacataggccaagtataaatgtacaatcacagtgaactaaagccataaaatctagttccctgacccttcaatcaaccattcagagcaatgggaatatagcggggagacagaagtcccactttggttgctcatattacattaagccagcctgccccaccccaatccccttcccaccaataaaaaagtcaccgtgagtgtataattggtcaatccagtttatccaaggtctatagatatagccatgatttgtcctatattcatgttaaatagaatgcttacataaaattaatactcaaagacattgagctgatgtgcatgtatattcttatttaacatttaagtggctttaatggtattttagaatgtcacctatggcatgagtcttcaaatctggattgaagactgtggcggttttataactgcatgtaagatcttaaatgtaagactctgggcctacctacattaaggcaggtgacagtaccctcattcattctacataataaatacactcttctgtgactgcaaaattctgaatccttgaatgatttactataataggctaaggttgtataaggcacttttggctctgaaatatttctcctaactctcaggctgaatcttaaagaaatatttacaaagctgcaacaaattaattttagaaccggatgctttattcgtaggtctaatggggatggtgagaagcaatttgtacacaatgcccattaatctctcactgtgccatgtatcaatcatagagaagatcccaggcatgggccacctgaactactatgtcgcttacttgacttctcaacagccacatgcccctttctccttttcttcacttaactgatccgtagaggcatgaccatttgatcgcaccactccttcaggaatccaggacttgtccacacaccgttccattcgcttcattatcaggtccagaagcatctcaattgcttggcttatgtttgtcccattggcagcactagtttcaaagtaggggattccatatttctctgcgagtgctatggcttcctcctctttcactactctctggtcctccagatcactcttgtttccacacagcactatatctgggttttcacaatatgcatgcatctgtagctggcttatccagtttctgacattgaggaaactttgctcatttgtcagatcaaaaagtagaagaaaacccatagcatctctgaagaacgctgtcgttaagctacgaaacctctcctgccctgctgtgtcccataactgcaggtggattctctggcctctgccagtggctccatccggcccactggctctgtacaccactcttttttccctgaaatcaatgcccactgttgtgataaatttggagttaaatttaccatctgtatattggtaaagtacactggtcttccctacaccagagtctcccaaagctaaaaacttgatgaggtaatcataatctccatcagacataatgaagaactcagtagttcaccttaccaaggacatgaacccttcacatttccatctgagttcctcaaaaaccatatggggattcttattggaattgcattgcattgcattgggatcacataaatctttacagggtagagaaccgcttgttatgattttctaaaacgttagagactggagttaccaatgcttcaacaattgacaacttccaatcacatgtcctcttcaggaaggttactttttgtctggctcgccccgccgtcctgtccccgcctggctcgggtcctcgcgcgccgcgtccacccgccgccggcctttttt

SEQ ID NO: 11203 - RNA, 3172 nt, Homo sapiens
  source 1..3172: mol_type = other RNA
ctgaatagctgggactacaggtgcccaccaccacgcccagcccattttttttttttttttttttttagtagagatggggtttcactgtgttagccaggatggtctcgatctcctgacctcgtgatccgccctcctcggcctcccaaagtgctgggattacaggtgtgagccaccgcgcctggccaaccctgctcttgaaatgtctaaatcttttcctcactagcatatacaattcaaatgcacaggcctccatgacttctttggaatttaaaagaagccttcatttcaaggatagaaatatgtaaaattttaccaaccatggataagtttgttatgggagtagtggaaggacagtggaaaaaaaaataggttttttcatgatacttttatttttccttttttaaaaataaatttagggggtacaagtacagtttagatacatgaatatattgtgtagtcgtaaagtctgggcttctagtgtaaccatcacgcaaatatacttgtatttttctaattacagttctaccaaacatttgccaccacaaaatacaagtatttttattctttatttaaattatggtgagtgatatttcttcctatatagccattaagatctctggaagttttgatctactttattcaaaccactttaataaataagacttttcacctaaatgaaatacctttgaattttataaacaacttccatgaaacatatattaaaaccacctttaatttggtatgaagacactttggcaatgcagcggaataaatgatcttggcaagacccagcaagtacagtaaatgctcatgagctctatgaaaaatataggctacagaatacttcatttttcttttattgaactacagtacaaatgtgactgcttcaatatgaacatctatcttccaccaaatagcaaacaggcatcttatgtaattaaaaactaattatttcaattccaccaatggaaaagcaaaacaagttgcaaatatcaacaatacagagcctgctggtaaagatagagatgagtaagttataagctaataaagctgcagcctgaggatgccagatcaacattataaatatgaagaaaaagaaactaaatatttactcatcgcaaataactcggcataagcaccagctatgttcaggtgcggccagcacataggccaagtataaatgtacaatcacagtgaactaaagccataaaatctagttccctgacccttcaatcaaccattcagagcaatgggaatatagcggggagacagaagtcccactttggttgctcatattacattaagccagcctgccccaccccaatccccttcccaccaataaaaaagtcaccgtgagtgtataattggtcaatccagtttatccaaggtctatagatatagccatgatttgtcctatattcatgttaaatagaatgcttacataaaattaatactcaaagacattgagctgatgtgcatgtatattcttatttaacatttaagtggctttaatggtattttagaatgtcacctatggcatgagtcttcaaatctggattgaagactgtggcggttttataactgcatgtaagatcttaaatgtaagactctgggcctacctacattaaggcaggtgacagtaccctcattcattctacataataaatacactcttctgtgactgcaaaattctgaatccttgaatgatttactataataggctaaggttgtataaggcacttttggctctgaaatatttctcctaactctcaggctgaatcttaaagaaatatttacaaagctgcaacaaattaattttagaaccggatgctttattcgtaggtctaatggggatggtgagaagcaatttgtacacaatgcccattaatctctcactgtgccatgtatcaatcatagagaagatcccaggcatgggccacctgaactactatgtcgcttacttgacttctcaacagccacatgcccctttctccttttcttcacttaactgatccgtagaggcatgaccatttgatcgcaccactccttcaggaatccaggacttgtccacacaccgttccattcgcttcattatcaggtccagaagcatctcaattgcttggcttatgtttgtcccattggcagcactagtttcaaagtaggggattccatatttctctgcgagtgctatggcttcctcctctttcactactctctggtcctccagatcactcttgtttccacacagcactatatctgggttttcacaatatgcatgcatctgtagctggcttatccagtttctgacattgaggaaactttgctcatttgtcagatcaaaaagtagaagaaaacccatagcatctctgaagaacgctgtcgttaagctacgaaacctctcctgccctgctgtgtcccataactgcaggtggattctctggcctctgccagtggctccatccggcccactggctctgtacaccactcttttttccctgaaatcaatgcccactgttgtgataaatttggagttaaatttaccatctgtatattggtaaagtacactggtcttccctacaccagagtctcccaaagctaaaaacttgatgaggtaatcataatctccatcagacataatgaagaactcagtagttcaccttatgctgaaaactcctgaatgctgagccccaaaagccactgcagtgtgtttcctcagagtgcttcagtgcagatctgcaacctcacgtttcaggtatggctagcccgtggataagggcagagcctcaagtcaagcagagctgggtttgaatcccaaatctcccagataccaattacttggatgtctttgagccttagatttccaggtttctgttcttaccaaggacatgaacccttcacatttccatctgagttcctcaaaaaccatatggggattcttattggaattgcattgcattgcattgggatcacataaatctttacagggtagagaaccgcttgttatgattttctaaaacgttagagactggagttaccaatgcttcaacaattgacaacttccaatcacatgtcctcttcaggaaggttactttttgtctggctcgccccgccgtcctgtccccgcctggctcgggtcctcgcgcgccgcgtccacccgccgccggcctttttt

SEQ ID NO: 11204 - RNA, 3091 nt, Homo sapiens
  source 1..3091: mol_type = other RNA
ctgaatagctgggactacaggtgcccaccaccacgcccagcccattttttttttttttttttttttagtagagatggggtttcactgtgttagccaggatggtctcgatctcctgacctcgtgatccgccctcctcggcctcccaaagtgctgggattacaggtgtgagccaccgcgcctggccaaccctgctcttgaaatgtctaaatcttttcctcactagcatatacaattcaaatgcacaggcctccatgacttctttggaatttaaaagaagccttcatttcaaggatagaaatatgtaaaattttaccaaccatggataagtttgttatgggagtagtggaaggacagtggaaaaaaaaataggttttttcatgatacttttatttttccttttttaaaaataaatttagggggtacaagtacagtttagatacatgaatatattgtgtagtcgtaaagtctgggcttctagtgtaaccatcacgcaaatatacttgtatttttctaattacagttctaccaaacatttgccaccacaaaatacaagtatttttattctttatttaaattatggtgagtgatatttcttcctatatagccattaagatctctggaagttttgatctactttattcaaaccactttaataaataagacttttcacctaaatgaaatacctttgaattttataaacaacttccatgaaacatatattaaaaccacctttaatttggtatgaagacactttggcaatgcagcggaataaatgatcttggcaagacccagcaagtacagtaaatgctcatgagctctatgaaaaatataggctacagaatacttcatttttcttttattgaactacagtacaaatgtgactgcttcaatatgaacatctatcttccaccaaatagcaaacaggcatcttatgtaattaaaaactaattatttcaattccaccaatggaaaagcaaaacaagttgcaaatatcaacaatacagagcctgctggtaaagatagagatgagtaagttataagctaataaagctgcagcctgaggatgccagatcaacattataaatatgaagaaaaagaaactaaatatttactcatcgcaaataactcggcataagcaccagctatgttcaggtgcggccagcacataggccaagtataaatgtacaatcacagtgaactaaagccataaaatctagttccctgacccttcaatcaaccattcagagcaatgggaatatagcggggagacagaagtcccactttggttgctcatattacattaagccagcctgccccaccccaatccccttcccaccaataaaaaagtcaccgtgagtgtataattggtcaatccagtttatccaaggtctatagatatagccatgatttgtcctatattcatgttaaatagaatgcttacataaaattaatactcaaagacattgagctgatgtgcatgtatattcttatttaacatttaagtggctttaatggtattttagaatgtcacctatggcatgagtcttcaaatctggattgaagactgtggcggttttataactgcatgtaagatcttaaatgtaagactctgggcctacctacattaaggcaggtgacagtaccctcattcattctacataataaatacactcttctgtgactgcaaaattctgaatccttgaatgatttactataataggctaaggttgtataaggcacttttggctctgaaatatttctcctaactctcaggctgaatcttaaagaaatatttacaaagctgcaacaaattaattttagaaccggatgctttattcgtaggtctaatggggatggtgagaagcaatttgtacacaatgcccattaatctctcactgtgccatgtatcaatcatagagaagatcccaggcatgggccacctgaactactatgtcgcttacttgacttctcaacagccacatgcccctttctccttttcttcacttaactgatccgtagaggcatgaccatttgatcgcaccactccttcaggaatccaggacttgtccacacaccgttccattcgcttcattatcaggtccagaagcatctcaattgcttggcttatgtttgtcccattggcagcactagtttcaaagtaggggattccatatttctctgcgagtgctatggcttcctcctctttcactactctctggtcctccagatcactcttgtttccacacagcactatatctgggttttcacaatatgcatgcatctgtagctggcttatccagtttctgacattgaggaaactttgctcatttgtcagatcaaaaagtagaagaaaacccatagcatctctgaagaacgctgtcgttaagctacgaaacctctcctgccctgctgtgtcccataactgcaggtggattctctggcctctgccagtggctccatccggcccactggctctgtacaccactcttttttccctgaaatcaatgcccactgttgtgataaatttggagttaaatttaccatctgtatattggtaaagtacactggtcttccctacaccagagtctcccaaagctaaaaacttgatgaggtaatcataatctccatcagacataatgaagaactcagtagttcaccttatgctgaaaactcctgaatgctgagccccaaaagccactgcagtgtgtttcctcagagtgcttcagtgcagatctgcaacctcacgtttcaggtatggctagcccgtggataagggcagagcctcaagtcaagcagagctgggtttgaatcccaaatctcccagataccaattacttggatgtctttgagccttagatttccaggtttctgttctttacagggtagagaaccgcttgttatgattttctaaaacgttagagactggagttaccaatgcttcaacaattgacaacttccaatcacatgtcctcttcaggaaggttactttttgtctggctcgccccgccgtcctgtccccgcctggctcgggtcctcgcgcgccgcgtccacccgccgccggccttttttgggtcgttggcgggtattttcc

SEQ ID NO: 11205 - RNA, 2892 nt, Homo sapiens
  source 1..2892: mol_type = other RNA
ctgaatagctgggactacaggtgcccaccaccacgcccagcccattttttttttttttttttttttagtagagatggggtttcactgtgttagccaggatggtctcgatctcctgacctcgtgatccgccctcctcggcctcccaaagtgctgggattacaggtgtgagccaccgcgcctggccaaccctgctcttgaaatgtctaaatcttttcctcactagcatatacaattcaaatgcacaggcctccatgacttctttggaatttaaaagaagccttcatttcaaggatagaaatatgtaaaattttaccaaccatggataagtttgttatgggagtagtggaaggacagtggaaaaaaaaataggttttttcatgatacttttatttttccttttttaaaaataaatttagggggtacaagtacagtttagatacatgaatatattgtgtagtcgtaaagtctgggcttctagtgtaaccatcacgcaaatatacttgtatttttctaattacagttctaccaaacatttgccaccacaaaatacaagtatttttattctttatttaaattatggtgagtgatatttcttcctatatagccattaagatctctggaagttttgatctactttattcaaaccactttaataaataagacttttcacctaaatgaaatacctttgaattttataaacaacttccatgaaacatatattaaaaccacctttaatttggtatgaagacactttggcaatgcagcggaataaatgatcttggcaagacccagcaagtacagtaaatgctcatgagctctatgaaaaatataggctacagaatacttcatttttcttttattgaactacagtacaaatgtgactgcttcaatatgaacatctatcttccaccaaatagcaaacaggcatcttatgtaattaaaaactaattatttcaattccaccaatggaaaagcaaaacaagttgcaaatatcaacaatacagagcctgctggtaaagatagagatgagtaagttataagctaataaagctgcagcctgaggatgccagatcaacattataaatatgaagaaaaagaaactaaatatttactcatcgcaaataactcggcataagcaccagctatgttcaggtgcggccagcacataggccaagtataaatgtacaatcacagtgaactaaagccataaaatctagttccctgacccttcaatcaaccattcagagcaatgggaatatagcggggagacagaagtcccactttggttgctcatattacattaagccagcctgccccaccccaatccccttcccaccaataaaaaagtcaccgtgagtgtataattggtcaatccagtttatccaaggtctatagatatagccatgatttgtcctatattcatgttaaatagaatgcttacataaaattaatactcaaagacattgagctgatgtgcatgtatattcttatttaacatttaagtggctttaatggtattttagaatgtcacctatggcatgagtcttcaaatctggattgaagactgtggcggttttataactgcatgtaagatcttaaatgtaagactctgggcctacctacattaaggcaggtgacagtaccctcattcattctacataataaatacactcttctgtgactgcaaaattctgaatccttgaatgatttactataataggctaaggttgtataaggcacttttggctctgaaatatttctcctaactctcaggctgaatcttaaagaaatatttacaaagctgcaacaaattaattttagaaccggatgctttattcgtaggtctaatggggatggtgagaagcaatttgtacacaatgcccattaatctctcactgtgccatgtatcaatcatagagaagatcccaggcatgggccacctgaactactatgtcgcttacttgacttctcaacagccacatgcccctttctccttttcttcacttaactgatccgtagaggcatgaccatttgatcgcaccactccttcaggaatccaggacttgtccacacaccgttccattcgcttcattatcaggtccagaagcatctcaattgcttggcttatgtttgtcccattggcagcactagtttcaaagtaggggattccatatttctctgcgagtgctatggcttcctcctctttcactactctctggtcctccagatcactcttgtttccacacagcactatatctgggttttcacaatatgcatgcatctgtagctggcttatccagtttctgacattgaggaaactttgctcatttgtcagatcaaaaagtagaagaaaacccatagcatctctgaagaacgctgtcgttaagctacgaaacctctcctgccctgctgtgtcccataactgcaggtggattctctggcctctgccagtggctccatccggcccactggctctgtacaccactcttttttccctgaaatcaatgcccactgttgtgataaatttggagttaaatttaccatctgtatattggtaaagtacactggtcttccctacaccagagtctcccaaagctaaaaacttgatgaggtaatcataatctccatcagacataatgaagaactcagtagttcacctttacagggtagagaaccgcttgttatgattttctaaaacgttagagactggagttaccaatgcttcaacaattgacaacttccaatcacatgtcctcttcaggaaggttactttttgtctaatgttaagacaaagagaaatgttaaagtcagaatggcctacttaaaaagtttttcaaaagagtctttggaaaagcagttcgctccatcaactttcaaaacaggcatcgctgt

SEQ ID NO: 11206 - RNA, 2841 nt, Homo sapiens
  source 1..2841: mol_type = other RNA
ctgaatagctgggactacaggtgcccaccaccacgcccagcccattttttttttttttttttttttagtagagatggggtttcactgtgttagccaggatggtctcgatctcctgacctcgtgatccgccctcctcggcctcccaaagtgctgggattacaggtgtgagccaccgcgcctggccaaccctgctcttgaaatgtctaaatcttttcctcactagcatatacaattcaaatgcacaggcctccatgacttctttggaatttaaaagaagccttcatttcaaggatagaaatatgtaaaattttaccaaccatggataagtttgttatgggagtagtggaaggacagtggaaaaaaaaataggttttttcatgatacttttatttttccttttttaaaaataaatttagggggtacaagtacagtttagatacatgaatatattgtgtagtcgtaaagtctgggcttctagtgtaaccatcacgcaaatatacttgtatttttctaattacagttctaccaaacatttgccaccacaaaatacaagtatttttattctttatttaaattatggtgagtgatatttcttcctatatagccattaagatctctggaagttttgatctactttattcaaaccactttaataaataagacttttcacctaaatgaaatacctttgaattttataaacaacttccatgaaacatatattaaaaccacctttaatttggtatgaagacactttggcaatgcagcggaataaatgatcttggcaagacccagcaagtacagtaaatgctcatgagctctatgaaaaatataggctacagaatacttcatttttcttttattgaactacagtacaaatgtgactgcttcaatatgaacatctatcttccaccaaatagcaaacaggcatcttatgtaattaaaaactaattatttcaattccaccaatggaaaagcaaaacaagttgcaaatatcaacaatacagagcctgctggtaaagatagagatgagtaagttataagctaataaagctgcagcctgaggatgccagatcaacattataaatatgaagaaaaagaaactaaatatttactcatcgcaaataactcggcataagcaccagctatgttcaggtgcggccagcacataggccaagtataaatgtacaatcacagtgaactaaagccataaaatctagttccctgacccttcaatcaaccattcagagcaatgggaatatagcggggagacagaagtcccactttggttgctcatattacattaagccagcctgccccaccccaatccccttcccaccaataaaaaagtcaccgtgagtgtataattggtcaatccagtttatccaaggtctatagatatagccatgatttgtcctatattcatgttaaatagaatgcttacataaaattaatactcaaagacattgagctgatgtgcatgtatattcttatttaacatttaagtggctttaatggtattttagaatgtcacctatggcatgagtcttcaaatctggattgaagactgtggcggttttataactgcatgtaagatcttaaatgtaagactctgggcctacctacattaaggcaggtgacagtaccctcattcattctacataataaatacactcttctgtgactgcaaaattctgaatccttgaatgatttactataataggctaaggttgtataaggcacttttggctctgaaatatttctcctaactctcaggctgaatcttaaagaaatatttacaaagctgcaacaaattaattttagaaccggatgctttattcgtaggtctaatggggatggtgagaagcaatttgtacacaatgcccattaatctctcactgtgccatgtatcaatcatagagaagatcccaggcatgggccacctgaactactatgtcgcttacttgacttctcaacagccacatgcccctttctccttttcttcacttaactgatccgtagaggcatgaccatttgatcgcaccactccttcaggaatccaggacttgtccacacaccgttccattcgcttcattatcaggtccagaagcatctcaattgcttggcttatgtttgtcccattggcagcactagtttcaaagtaggggattccatatttctctgcgagtgctatggcttcctcctctttcactactctctggtcctccagatcactcttgtttccacacagcactatatctgggttttcacaatatgcatgcatctgtagctggcttatccagtttctgacattgaggaaactttgctcatttgtcagatcaaaaagtagaagaaaacccatagcatctctgaagaacgctgtcgttaagctacgaaacctctcctgccctgctgtgtcccataactgcaggtggattctctggcctctgccagtggctccatccggcccactggctctgtacaccactcttttttccctgaaatcaatgcccactgttgtgataaatttggagttaaatttaccatctgtatattggtaaagtacactggtcttccctacaccagagtctcccaaagctaaaaacttgatgaggtaatcataatctccatcagacataatgaagaactcagtagttcacctttacagggtagagaaccgcttgttatgattttctaaaacgttagagactggagttaccaatgcttcaacaattgacaacttccaatcacatgtcctcttcaggaaggttactttttgtctcctttgcttttctccacaaccttgcttcaaacccacttctcttcctgtgtcttgaatcacac

SEQ ID NO: 11207 - RNA, 2875 nt, Homo sapiens
  source 1..2875: mol_type = other RNA
ctgaatagctgggactacaggtgcccaccaccacgcccagcccattttttttttttttttttttttagtagagatggggtttcactgtgttagccaggatggtctcgatctcctgacctcgtgatccgccctcctcggcctcccaaagtgctgggattacaggtgtgagccaccgcgcctggccaaccctgctcttgaaatgtctaaatcttttcctcactagcatatacaattcaaatgcacaggcctccatgacttctttggaatttaaaagaagccttcatttcaaggatagaaatatgtaaaattttaccaaccatggataagtttgttatgggagtagtggaaggacagtggaaaaaaaaataggttttttcatgatacttttatttttccttttttaaaaataaatttagggggtacaagtacagtttagatacatgaatatattgtgtagtcgtaaagtctgggcttctagtgtaaccatcacgcaaatatacttgtatttttctaattacagttctaccaaacatttgccaccacaaaatacaagtatttttattctttatttaaattatggtgagtgatatttcttcctatatagccattaagatctctggaagttttgatctactttattcaaaccactttaataaataagacttttcacctaaatgaaatacctttgaattttataaacaacttccatgaaacatatattaaaaccacctttaatttggtatgaagacactttggcaatgcagcggaataaatgatcttggcaagacccagcaagtacagtaaatgctcatgagctctatgaaaaatataggctacagaatacttcatttttcttttattgaactacagtacaaatgtgactgcttcaatatgaacatctatcttccaccaaatagcaaacaggcatcttatgtaattaaaaactaattatttcaattccaccaatggaaaagcaaaacaagttgcaaatatcaacaatacagagcctgctggtaaagatagagatgagtaagttataagctaataaagctgcagcctgaggatgccagatcaacattataaatatgaagaaaaagaaactaaatatttactcatcgcaaataactcggcataagcaccagctatgttcaggtgcggccagcacataggccaagtataaatgtacaatcacagtgaactaaagccataaaatctagttccctgacccttcaatcaaccattcagagcaatgggaatatagcggggagacagaagtcccactttggttgctcatattacattaagccagcctgccccaccccaatccccttcccaccaataaaaaagtcaccgtgagtgtataattggtcaatccagtttatccaaggtctatagatatagccatgatttgtcctatattcatgttaaatagaatgcttacataaaattaatactcaaagacattgagctgatgtgcatgtatattcttatttaacatttaagtggctttaatggtattttagaatgtcacctatggcatgagtcttcaaatctggattgaagactgtggcggttttataactgcatgtaagatcttaaatgtaagactctgggcctacctacattaaggcaggtgacagtaccctcattcattctacataataaatacactcttctgtgactgcaaaattctgaatccttgaatgatttactataataggctaaggttgtataaggcacttttggctctgaaatatttctcctaactctcaggctgaatcttaaagaaatatttacaaagctgcaacaaattaattttagaaccggatgctttattcgtaggtctaatggggatggtgagaagcaatttgtacacaatgcccattaatctctcactgtgccatgtatcaatcatagagaagatcccaggcatgggccacctgaactactatgtcgcttacttgacttctcaacagccacatgcccctttctccttttcttcacttaactgatccgtagaggcatgaccatttgatcgcaccactccttcaggaatccaggacttgtccacacaccgttccattcgcttcattatcaggtccagaagcatctcaattgcttggcttatgtttgtcccattggcagcactagtttcaaagtaggggattccatatttctctgcgagtgctatggcttcctcctctttcactactctctggtcctccagatcactcttgtttccacacagcactatatctgggttttcacaatatgcatgcatctgtagctggcttatccagtttctgacattgaggaaactttgctcatttgtcagatcaaaaagtagaagaaaacccatagcatctctgaagaacgctgtcgttaagctacgaaacctctcctgccctgctgtgtcccataactgcaggtggattctctggcctctgccagtggctccatccggcccactggctctgtacaccactcttttttccctgaaatcaatgcccactgttgtgataaatttggagttaaatttaccatctgtatattggtaaagtacactggtcttccctacaccagagtctcccaaagctaaaaacttgatgaggtaatcataatctccatcagacataatgaagaactcagtagttcacctttacagggtagagaaccgcttgttatgattttctaaaacgttagagactggagttaccaatgcttcaacaattgacaacttccaatcacatgtcctcttcaggaaggttactttttgtctggctcgccccgccgtcctgtccccgcctggctcgggtcctcgcgcgccgcgtccacccgccgccggccttttttgggtcgttggcgggtattttcc

SEQ ID NO: 11208 - RNA, 245 nt, Homo sapiens
  source 1..245: mol_type = other RNA
ctgaatagctgggactacaggtgcccaccaccacgcccagctaattttttgtacttttagtagagacagggttttaccgtgttagccaggatagtctcgatctcctgacctcgtgagccgcctgcctcggcctcccaaagtgctgggattacaggcatgagccaccgtgcctggccacgtccctattttagaaatgagaggagtgactgcacataggaaaaatgccacttttagcaattcaaagt

SEQ ID NO: 11209 - RNA, 1769 nt, Homo sapiens
  source 1..1769: mol_type = other RNA
ctgaatagctgggactacaggtgcccaccaccacgcccagctaattttttgtacttttagtagagacagggttttaccgtgttagccaggatagtctcgatctcctgacctcgtgagccgcctgcctcggcctcccaaagtgctgggattacaggcatgagccaccgtgcctggccacgtccctattttagaaatgagaggagtgactgcacataggaaaaatgccacttttagcaattcaaagtggaaaaacttcttttatataaaaattatcccaactcccaccccttggctctcagtgttgcatctcccacagaggtaaagttgtgccattttcccacggctttaaacaaagcaaaacaaaaccaccaatcctaataacccccctccttgccccgtctccacgctgtgcggagagggctctagcccctcagtcggacttctccttctccttcatgtgcaagaagacgatgctgaagatgaagagccccagcatcatggagaaggcgctggcgtagtaggggtaggccgaggggatgaagcgctcatactgcgtgtgctggagtggccgcacggatacctgagtggaagagtacaggtgtgtgtagcctagccggttgtaatccactttaaactggaatacaccatacacgtcgggcaacttgaactgaacactgtatttgccacctttcttcttcaggaaggtcctcacaaaaggatcaatgcggacaaactccagctgaatgtcatcgccatcaaaggggacccatttgccatttgagagctgctggatcacgatgctatactccactaggtcagtgacagtgtaggcattgggtggggctgtctcgcccacccgatgatgggacacaggccccacacggaggacaccctcctccttgaacacccagcgggagagggccacagctagttcatagttgcctgtctgggaatacctctgggagccgggcgccgccttctgcactgctgagttgaagaaggagtcgctgaagaagtcgagggagccgctgaagatgacgcgggcattgttcctggcctggagcccagcaatgaggagggtgttcttccccaccgcatgtggatactgggtgataggcttgtccgggaagaaggagtaagaggtggaagagcccgtcaggatgtccagcaccaaagggttatcaggatcggccaccatcccaacacctcgaaagaggatgggatttagagatgatttcccaacgatggttggggccttcagcaggttctcagtgtcagccacgatgagcgtatgctggccaaggtctgagatgtcatagttgtgatggtcaatgacagccgttttctcctcgtcaaactcaatcccgcactcactgcccagctctcgaagagggtcaccaatgtcggagctggcagctaccagcacactgcctccgccgtcaataaaggcactgatggtctccacgttgatgttgcctccaaaatcttctaccgaaggggagaaaatgatgagattgtcatagaggaattccccatactttatgagagacaggctggggtcatcagcggtcttgaatgtgagctcaaagccccggtccttcaggctccggaagaaaagcgaatgagtctcccgcacgttgaggttgtccagcagcactaaggtgcggggtccgctggcgcaaaccgcgccaagcaagggcagcagcaaccaaaagagggcccaagcccgggccgcggtgctgggctccatcttcctcctcctgccgaag

SEQ ID NO: 11210 - RNA, 2452 nt, Homo sapiens
  source 1..2452: mol_type = other RNA
ctgaatagctgggactacaggtgcccaccaccacgcccagctaattttttgtatttttagtagagacggagtttcaacgcattagccaggatggtctcgatctcctgaccttgtgatccacccgtctcggcctcccacagtgctgggattacatggatgagcaactgtgcccggccaacaaaaagcatttctataaaataacaataaaaaaagagttaaaaaagcaagcttccactttattaaaaagcaaaaattaccaactcgtataaaataatttaactcataaaaaggagaatcaaacattactttttaaaatatcagataccataaaatgtgcatttagtcttttaaatagttaaactttcagttaaactattaaacacctagcttttctcagaaagctgttgcaaacccaagtactgttctgactgtacagaaatcaatgatcctcttctttagcagaataaagatgtaactcccttaaatgacattcaccttaatattaccaacttaaattctgcttcattaccagaaacagtgttttcaagaactggatctttctaaatccacttttatttttacaacaactttactatttgattaaattcactgtagaaaaatgtgaagacacagaaagattcaaagaaaataaaaattatcccagtatccctcccccaaatacaataacaaggttatatatatttctttctagtttttttgtatatttacatagcattttaaagcaaaactagtactataaaatgctaccatatccttttttcacttcatatatagagcaaccgtgtctttttaggacattgaaatatgcaaaaaggattttcagttggctgattcacaatctaattataactaagacataatttacctccaattgcaagggattcagattgtttcaattatttattattataactatcattattaaacacccttctttatatataattctttgtatgcatctctgatatggttttaaagagaaattgctagatgtagagttcccagcacaaagtacgtccgtatttttaagtcttttgatgcattttaccaaattgccctccagaaatactgtaccaatttacagtcgcatcaataaataaccaaagagtcccatttcttcctcacattctttggcagtataggaaagtagagattaccctccaccctttattgttgcaaatttaatagggggagaagagaatggtgggtttttttttcccccttaaaatgtaatattttttcccacatgtttactagtcatttgcttttcttctgtattttgaagttgtctaaatcattcaggagtctctaatacacacaatgtcttgtctttcttacaacatactctttgataggcaagggcatgaaagctgcatgtctttcccatatttttttcaagttaagcaggaattcccaaaatgactggaattagaatgtcttcttttctcctgggcagccatgctactttaatgtcttggtaataaaacagaaaactgggccatattcttcaggttatggagggtttctgaccattctgtggaccctatctgaggtatggtagtgagcagtaagcttttggctttattagcgttttctttcagggtctttaagacccggtccaccgaaactgcttcctcgtgctccttccagcagtcataatctgtcgccatggcgatacttgcgtaacaaattccagcctccttagcaagaaccacctctggaactgtggtcatgttgataacatccgccccccaggtgcggaacatgaagctttctgcccgggagctaaaacgaggtccctcgattgtgaccattgtcccctttgagtggcaccggagtcctagcttcttagcagtctctataagaacctctctcgttttggggcaaaacggctcagccattggaatatggcacactcctctggcacaagaatgacttccatcatagaaggactgaggtctcatagtggtcctgtcaatgaactgatcaataatgacaatatcgccgggctgaatctcctccctcaaggagccacaagctgtggtcactatgacatgtgtacagccctcttccttcaaagcccagatgttcgcctggtagttgacctttgaaggcatgatggtgtgctgccttccatgccttgcaaggaggacgcaatcaacattttttatcttccccaaaattaaggcatcagatggcttgccaaatggagtatccacatatttttcagttcttccttctaaaatttctggatcatccaggcctgttccaccaattattccaatcttcacggcggtggtggtggtgccagaggccatgtctgcacgggaaaggaatctgcagtgggcgagcgctcgggactaagggaaccaagcgagccacagagcggtggctgtgccaacctcactgcgcgggagtgagcagtgcggag

SEQ ID NO: 11211 - RNA, 4463 nt, Homo sapiens
  source 1..4463: mol_type = other RNA
ctgaatagctgggactacaggtgcccaccaccacgcccagctaatttttttttgtatttttagtagagacggggtttcactgttagccaggatggtctggatctcctgacctcgtgatctgcccatctcagccacccacaaagtgctgggattagaggcgtgggccaccacgcccagcctgcaatcttttcaattactaacacttgatccaaatgtaaagcagcaaatagattaaaagaaaacaaacaaaccaaggcattacttaaggtgtttttccaaaaatccaattcctggagctagatgtataaaaagcataaaaacaaaattatcaacaactaggttaattgttaggtgaagtagtcacaaaaaacatcccagggagaaaggttaggtttatgtaacatgatgtaatggaaacatcactagacagtaaaccagataacctggatcccactcccatgagacataactggttatatgtacttggcctcatagctatctacatttctatttctgcaaggaacttagaaaactggagggtttagaccagatgctttctaaggttatcttacaatttaaactgttacaattttaagtcttctgagaaacatttgttatcagccgtaacaggaatgttataattagatggaatgtgagttgctaggaacacaggtatgcacatacaacaaaatagtggggataaaaataataccttctaagaatacttgcagccaccattgtccaaacagactaaattcttgaagtgggaaaatcattggtcataaattgatcttccacttatatcaataaacctaaaaaataatgttagcagtgcttgttaaatttgagggcaatgatacatataattctatcttctttatagtgctgtttcagactctgctactcaattgtgttccctcccaaattcatatgttgaagtcctaaacctcagcaccttagaatatgaccttatttggagatcaggtctttaagttaaaaggaggacattgggaggggccctaatccaatcaatatgactggagtctttataaaaacaagaaatttggcctggggcggtgcctcatgcctgtaatcccagcactttgggagactgaggcaggtggatcacctgaggtcaggaatttgagaccagcctggccaacgtggtgaaaccccgtttctactaaaaatacaaaattagcctggcatggtggctgacgcctgttaaccccagctacttgggaagctgaggcagcagaatcacttgaacctgggaggcggaggttgcaatgagctgagatcgcgccactgtactccagcctgggcgacaagagtgaaattctgtctcaaaaaattaaaaaagcaaaaaaaaaaaaaaaaagaggaaatttgggggacagacttgcacacagggagaacaccatgtgaacatgaggctatccatctacaagccaaggacagacctgaaacagatccttcccccacaaccctcagaaggaaccaactgccaataactccattttgaatgtctggccttcacaactgtgagaccataaatttctgctaggtaggcaactcagtttgtagtaatttgttatggcagccatacgaactaatattgatgctaatttatcattttattaataaatgttgtaagttatacattttcatgccagcaacccctatctcccagatcttcctaactttaaatacttcagtgggttttctgtcaatgaacaatttgacatcagaaatttgggcaagagtcaggcataatggctcatgcctataatcccagtgatttggaaggccaaggtgggaggattgcttgagtccaggagtttgagactggcctgggcaacatagcgagatctcatctctacaagaaatttaaaaacttagcgggcatggtgccacatgcctgtagtcctagctatgcaggagggtgaagtgggaggattgctcgagcctgggagactacagcccgggagctatgatcaaccactgcactccatcctggacaacagaacgagaccatctctaagaaaaaaatattaagtctgtgaatgaatttatggttcctcaacagaaaatgaaacatcaagttatgaatgagttatgatatagttattttttattgtgtaagcccttattagttcctccctcatcccatcttaaaatattcaacaatagatagtggctcaaaaatttttttttaaaaaaacagactgccatgaaaaccaaatcttttcttcctgtaatagtggcttcctagtgttatttctcattaatgggagtatccgtggacttaactgtatattgcattttagttctggtcgtgtaataatttaatgacttcacacataaaaaactaatcttgtcttgagttttaaaaagttactagcacccatggttaaggaaggaaaactgtagctcacttcttcaatacatttgtttcttttcaattcatgaaatcagagaatatggaagaaacaggatgacagtcaccaagagtggttgaaactacaaactatcacgcaattgaaaataccacattaaagatatatttatatacagaaaatggagcaatgccaataaaattttataatttaaaaaagttacttgttaaaggcagatttcataagttgtgtttacaatcatccatttaatcatctccaaaaaaaggatgaatttattattttaaactaacattctgtaagttaaagagaataatcaagttgtctcatggactggaaggtgacttattaattccctttcatttccaaacctcatcaagcagtcactacatttatgaggcaagtcagctgaatgcttgaaatctagatgaattttaagatcttcaatttgtcctgttgaatattcacaatattgacataaataaatcccttcagataaatgtgaatttaaatgcttgcaatattctagcatacttgaaaagcctttcccacagtcatcacaaacatgaggaaaaatttttgtatgttcaatagcaacatgcctgttaacatttgtgtgaagtctactccgaaaaccacatacttgacatacaaagaagtttttacatttgtcaaaggtaattttgcttaagaggctatactgtccatgttcaccattgttatacttatcacttaactctattaatttacatgcatgctcatttaccacatggctatgcaagtcttctggatcattagtttcatgttcacagaactgacacaagtactgttcatcacagctgtgctcctggaaatgtaggtagagttcactgcttgaggagaactgtacatcacactgttcacaccaatagaggtgatcactaaaatgggtgtctgcaatgtgctggctgaggttctcaaaaattactgtcttataatcacagtatttacaaatgtagggatcctcttcatgcagtttggcatgttctatcagaagcatattggtagagaaactttccttgcatactcgacacacatttgaatcagtacgtttatgcttcaggatcatatgctgctttaagtcagaaaaatatttgctgttaaactcacaaagttcacatttatagaggccactgctattagctctcagtaaaggccatttctgctgggcagtcacattcaaagcttggctcttgtcaagaattttacaaagtttagctggcggttcttcatcagtttggtcttggagactctcagaggaattgttttctgtctctatatcataatcctcagaaatcgcatgcacttctacagcaattggaacatcttcagcagtgtgaacttctataggactctcctcttgggtttgctggttgactgattcaggtgagtcacactcttcatcacaaattacaatatcagcagatttttctgtagaaaaggcagtgtggtctagaattctaagtacaggactgggaaccaggtagttctgatttctgtttctggccttgattccatctgcaaattttggcaagtcatttgacgtctcggtatcagaatcatcatctttgttgtcaaaatattttaaatctggctgtctcatagaacagacactgtaacaatgatcagagaaaattccattgaatccatctgcaattctgcttattccagaggaatctgaataacgagaagggtgtagagtcttcctttttctttttttaggatactcattcatatcttttcaatcagtcagtcccccgaggccctcccggccggcccacgcagaggcggcggcggccgagagcgcaggcggaggggccgcgcggtccttcccgcggacgcacggcggcgggcagcgctgctccggccctagcgctcccggacgctgtgctgggccgacccctctccctccccgcgcgccccacgccctgagcgccaggcccctggcctaggctccgcggccgcactgccctggccgccacgctccgcgcctgcgccgcgcacctc

SEQ ID NO: 11212 - RNA, 4414 nt, Homo sapiens
  source 1..4414: mol_type = other RNA
ctgaatagctgggactacaggtgcccaccaccacgcccagctaatttttttttgtatttttagtagagacggggtttcactgttagccaggatggtctggatctcctgacctcgtgatctgcccatctcagccacccacaaagtgctgggattagaggcgtgggccaccacgcccagcctgcaatcttttcaattactaacacttgatccaaatgtaaagcagcaaatagattaaaagaaaacaaacaaaccaaggcattacttaaggtgtttttccaaaaatccaattcctggagctagatgtataaaaagcataaaaacaaaattatcaacaactaggttaattgttaggtgaagtagtcacaaaaaacatcccagggagaaaggttaggtttatgtaacatgatgtaatggaaacatcactagacagtaaaccagataacctggatcccactcccatgagacataactggttatatgtacttggcctcatagctatctacatttctatttctgcaaggaacttagaaaactggagggtttagaccagatgctttctaaggttatcttacaatttaaactgttacaattttaagtcttctgagaaacatttgttatcagccgtaacaggaatgttataattagatggaatgtgagttgctaggaacacaggtatgcacatacaacaaaatagtggggataaaaataataccttctaagaatacttgcagccaccattgtccaaacagactaaattcttgaagtgggaaaatcattggtcataaattgatcttccacttatatcaataaacctaaaaaataatgttagcagtgcttgttaaatttgagggcaatgatacatataattctatcttctttatagtgctgtttcagactctgctactcaattgtgttccctcccaaattcatatgttgaagtcctaaacctcagcaccttagaatatgaccttatttggagatcaggtctttaagttaaaaggaggacattgggaggggccctaatccaatcaatatgactggagtctttataaaaacaagaaatttggcctggggcggtgcctcatgcctgtaatcccagcactttgggagactgaggcaggtggatcacctgaggtcaggaatttgagaccagcctggccaacgtggtgaaaccccgtttctactaaaaatacaaaattagcctggcatggtggctgacgcctgttaaccccagctacttgggaagctgaggcagcagaatcacttgaacctgggaggcggaggttgcaatgagctgagatcgcgccactgtactccagcctgggcgacaagagtgaaattctgtctcaaaaaattaaaaaagcaaaaaaaaaaaaaaaaagaggaaatttgggggacagacttgcacacagggagaacaccatgtgaacatgaggctatccatctacaagccaaggacagacctgaaacagatccttcccccacaaccctcagaaggaaccaactgccaataactccattttgaatgtctggccttcacaactgtgagaccataaatttctgctaggtaggcaactcagtttgtagtaatttgttatggcagccatacgaactaatattgatgctaatttatcattttattaataaatgttgtaagttatacattttcatgccagcaacccctatctcccagatcttcctaactttaaatacttcagtgggttttctgtcaatgaacaatttgacatcagaaatttgggcaagagtcaggcataatggctcatgcctataatcccagtgatttggaaggccaaggtgggaggattgcttgagtccaggagtttgagactggcctgggcaacatagcgagatctcatctctacaagaaatttaaaaacttagcgggcatggtgccacatgcctgtagtcctagctatgcaggagggtgaagtgggaggattgctcgagcctgggagactacagcccgggagctatgatcaaccactgcactccatcctggacaacagaacgagaccatctctaagaaaaaaatattaagtctgtgaatgaatttatggttcctcaacagaaaatgaaacatcaagttatgaatgagttatgatatagttattttttattgtgtaagcccttattagttcctccctcatcccatcttaaaatattcaacaatagatagtggctcaaaaatttttttttaaaaaaacagactgccatgaaaaccaaatcttttcttcctgtaatagtggcttcctagtgttatttctcattaatgggagtatccgtggacttaactgtatattgcattttagttctggtcgtgtaataatttaatgacttcacacataaaaaactaatcttgtcttgagttttaaaaagttactagcacccatggttaaggaaggaaaactgtagctcacttcttcaatacatttgtttcttttcaattcatgaaatcagagaatatggaagaaacaggatgacagtcaccaagagtggttgaaactacaaactatcacgcaattgaaaataccacattaaagatatatttatatacagaaaatggagcaatgccaataaaattttataatttaaaaaagttacttgttaaaggcagatttcataagttgtgtttacaatcatccatttaatcatctccaaaaaaaggatgaatttattattttaaactaacattctgtaagttaaagagaataatcaagttgtctcatggactggaaggtgacttattaattccctttcatttccaaacctcatcaagcagtcactacatttatgaggcaagtcagctgaatgcttgaaatctagatgaattttaagatcttcaatttgtcctgttgaatattcacaatattgacataaataaatcccttcagataaatgtgaatttaaatgcttgcaatattctagcatacttgaaaagcctttcccacagtcatcacaaacatgaggaaaaatttttgtatgttcaatagcaacatgcctgttaacatttgtgtgaagtctactccgaaaaccacatacttgacatacaaagaagtttttacatttgtcaaaggtaattttgcttaagaggctatactgtccatgttcaccattgttatacttatcacttaactctattaatttacatgcatgctcatttaccacatggctatgcaagtcttctggatcattagtttcatgttcacagaactgacacaagtactgttcatcacagctgtgctcctggaaatgtaggtagagttcactgcttgaggagaactgtacatcacactgttcacaccaatagaggtgatcactaaaatgggtgtctgcaatgtgctggctgaggttctcaaaaattactgtcttataatcacagtatttacaaatgtagggatcctcttcatgcagtttggcatgttctatcagaagcatattggtagagaaactttccttgcatactcgacacacatttgaatcagtacgtttatgcttcaggatcatatgctgctttaagtcagaaaaatatttgctgttaaactcacaaagttcacatttatagaggccactgctattagctctcagtaaaggccatttctgctgggcagtcacattcaaagcttggctcttgtcaagaattttacaaagtttagctggcggttcttcatcagtttggtcttggagactctcagaggaattgttttctgtctctatatcataatcctcagaaatcgcatgcacttctacagcaattggaacatcttcagcagtgtgaacttctataggactctcctcttgggtttgctggttgactgattcaggtgagtcacactcttcatcacaaattacaatatcagcagatttttctgtagaaaaggcagtgtggtctagaattctaagtacaggactgggaaccaggtagttctgatttctgtttctggccttgattccatctgcaaattttggcaagtcatttgacgtctcggtatcagaatcatcatctttgttgtcaaaatattttaaatctggctgtctcatagaacagacactgtaacaatgatcagagaaaattccattgaatccatctgcaattctgcttattccagaggaatctgaataacgagaagggtgtagagtcttcctttttctttttttaggatactcattcatatcttttcaatttggtataattcttactactggagtgaggaaaaatgaattacaataagtttctgtagacagtaaaaaatgccagcttcgcccgggcccagaagccggcgccaaggagacttccaagccccgacaccaaaggttccgtaaagacaacggcagcagggggccgaggggagcccggccaaggcgtcctgcgcagggggtggaactgccttcggga

SEQ ID NO: 11213 - RNA, 4534 nt, Homo sapiens
  source 1..4534: mol_type = other RNA
ctgaatagctgggactacaggtgcccaccaccacgcccagctaatttttttttgtatttttagtagagacggggtttcactgttagccaggatggtctggatctcctgacctcgtgatctgcccatctcagccacccacaaagtgctgggattagaggcgtgggccaccacgcccagcctgcaatcttttcaattactaacacttgatccaaatgtaaagcagcaaatagattaaaagaaaacaaacaaaccaaggcattacttaaggtgtttttccaaaaatccaattcctggagctagatgtataaaaagcataaaaacaaaattatcaacaactaggttaattgttaggtgaagtagtcacaaaaaacatcccagggagaaaggttaggtttatgtaacatgatgtaatggaaacatcactagacagtaaaccagataacctggatcccactcccatgagacataactggttatatgtacttggcctcatagctatctacatttctatttctgcaaggaacttagaaaactggagggtttagaccagatgctttctaaggttatcttacaatttaaactgttacaattttaagtcttctgagaaacatttgttatcagccgtaacaggaatgttataattagatggaatgtgagttgctaggaacacaggtatgcacatacaacaaaatagtggggataaaaataataccttctaagaatacttgcagccaccattgtccaaacagactaaattcttgaagtgggaaaatcattggtcataaattgatcttccacttatatcaataaacctaaaaaataatgttagcagtgcttgttaaatttgagggcaatgatacatataattctatcttctttatagtgctgtttcagactctgctactcaattgtgttccctcccaaattcatatgttgaagtcctaaacctcagcaccttagaatatgaccttatttggagatcaggtctttaagttaaaaggaggacattgggaggggccctaatccaatcaatatgactggagtctttataaaaacaagaaatttggcctggggcggtgcctcatgcctgtaatcccagcactttgggagactgaggcaggtggatcacctgaggtcaggaatttgagaccagcctggccaacgtggtgaaaccccgtttctactaaaaatacaaaattagcctggcatggtggctgacgcctgttaaccccagctacttgggaagctgaggcagcagaatcacttgaacctgggaggcggaggttgcaatgagctgagatcgcgccactgtactccagcctgggcgacaagagtgaaattctgtctcaaaaaattaaaaaagcaaaaaaaaaaaaaaaaagaggaaatttgggggacagacttgcacacagggagaacaccatgtgaacatgaggctatccatctacaagccaaggacagacctgaaacagatccttcccccacaaccctcagaaggaaccaactgccaataactccattttgaatgtctggccttcacaactgtgagaccataaatttctgctaggtaggcaactcagtttgtagtaatttgttatggcagccatacgaactaatattgatgctaatttatcattttattaataaatgttgtaagttatacattttcatgccagcaacccctatctcccagatcttcctaactttaaatacttcagtgggttttctgtcaatgaacaatttgacatcagaaatttgggcaagagtcaggcataatggctcatgcctataatcccagtgatttggaaggccaaggtgggaggattgcttgagtccaggagtttgagactggcctgggcaacatagcgagatctcatctctacaagaaatttaaaaacttagcgggcatggtgccacatgcctgtagtcctagctatgcaggagggtgaagtgggaggattgctcgagcctgggagactacagcccgggagctatgatcaaccactgcactccatcctggacaacagaacgagaccatctctaagaaaaaaatattaagtctgtgaatgaatttatggttcctcaacagaaaatgaaacatcaagttatgaatgagttatgatatagttattttttattgtgtaagcccttattagttcctccctcatcccatcttaaaatattcaacaatagatagtggctcaaaaatttttttttaaaaaaacagactgccatgaaaaccaaatcttttcttcctgtaatagtggcttcctagtgttatttctcattaatgggagtatccgtggacttaactgtatattgcattttagttctggtcgtgtaataatttaatgacttcacacataaaaaactaatcttgtcttgagttttaaaaagttactagcacccatggttaaggaaggaaaactgtagctcacttcttcaatacatttgtttcttttcaattcatgaaatcagagaatatggaagaaacaggatgacagtcaccaagagtggttgaaactacaaactatcacgcaattgaaaataccacattaaagatatatttatatacagaaaatggagcaatgccaataaaattttataatttaaaaaagttacttgttaaaggcagatttcataagttgtgtttacaatcatccatttaatcatctccaaaaaaaggatgaatttattattttaaactaacattctgtaagttaaagagaataatcaagttgtctcatggactggaaggtgacttattaattccctttcatttccaaacctcatcaagcagtcactacatttatgaggcaagtcagctgaatgcttgaaatctagatgaattttaagatcttcaatttgtcctgttgaatattcacaatattgacataaataaatcccttcagataaatgtgaatttaaatgcttgcaatattctagcatacttgaaaagcctttcccacagtcatcacaaacatgaggaaaaatttttgtatgttcaatagcaacatgcctgttaacatttgtgtgaagtctactccgaaaaccacatacttgacatacaaagaagtttttacatttgtcaaaggtaattttgcttaagaggctatactgtccatgttcaccattgttatacttatcacttaactctattaatttacatgcatgctcatttaccacatggctatgcaagtcttctggatcattagtttcatgttcacagaactgacacaagtactgttcatcacagctgtgctcctggaaatgtaggtagagttcactgcttgaggagaactgtacatcacactgttcacaccaatagaggtgatcactaaaatgggtgtctgcaatgtgctggctgaggttctcaaaaattactgtcttataatcacagtatttacaaatgtagggatcctcttcatgcagtttggcatgttctatcagaagcatattggtagagaaactttccttgcatactcgacacacatttgaatcagtacgtttatgcttcaggatcatatgctgctttaagtcagaaaaatatttgctgttaaactcacaaagttcacatttatagaggccactgctattagctctcagtaaaggccatttctgctgggcagtcacattcaaagcttggctcttgtcaagaattttacaaagtttagctggcggttcttcatcagtttggtcttggagactctcagaggaattgttttctgtctctatatcataatcctcagaaatcgcatgcacttctacagcaattggaacatcttcagcagtgtgaacttctataggactctcctcttgggtttgctggttgactgattcaggtgagtcacactcttcatcacaaattacaatatcagcagatttttctgtagaaaaggcagtgtggtctagaattctaagtacaggactgggaaccaggtagttctgatttctgtttctggccttgattccatctgcaaattttggcaagtcatttgacgtctcggtatcagaatcatcatctttgttgtcaaaatattttaaatctggctgtctcatagaacagacactgtaacaatgatcagagaaaattccattgaatccatctgcaattctgcttattccagaggaatctgaataacgagaagggtgtagagtcttcctttttctttttttaggatactcattcatatcttttcaatttggtataattcttactactggagtgaggaaaaatgaattacaataagtttctgtagacagtaaaaaatgccagtcagtcccccgaggccctcccggccggcccacgcagaggcggcggcggccgagagcgcaggcggaggggccgcgcggtccttcccgcggacgcacggcggcgggcagcgctgctccggccctagcgctcccggacgctgtgctgggccgacccctctccctccccgcgcgccccacgccctgagcgccaggcccctggcctaggctccgcggccgcactgccctggccgccacgctccgcgcctgcgccgcgcacctc

SEQ ID NO: 11214 - RNA, 4578 nt, Homo sapiens
  source 1..4578: mol_type = other RNA
ctgaatagctgggactacaggtgcccaccaccacgcccagctaatttttttttgtatttttagtagagacggggtttcactgttagccaggatggtctggatctcctgacctcgtgatctgcccatctcagccacccacaaagtgctgggattagaggcgtgggccaccacgcccagcctgcaatcttttcaattactaacacttgatccaaatgtaaagcagcaaatagattaaaagaaaacaaacaaaccaaggcattacttaaggtgtttttccaaaaatccaattcctggagctagatgtataaaaagcataaaaacaaaattatcaacaactaggttaattgttaggtgaagtagtcacaaaaaacatcccagggagaaaggttaggtttatgtaacatgatgtaatggaaacatcactagacagtaaaccagataacctggatcccactcccatgagacataactggttatatgtacttggcctcatagctatctacatttctatttctgcaaggaacttagaaaactggagggtttagaccagatgctttctaaggttatcttacaatttaaactgttacaattttaagtcttctgagaaacatttgttatcagccgtaacaggaatgttataattagatggaatgtgagttgctaggaacacaggtatgcacatacaacaaaatagtggggataaaaataataccttctaagaatacttgcagccaccattgtccaaacagactaaattcttgaagtgggaaaatcattggtcataaattgatcttccacttatatcaataaacctaaaaaataatgttagcagtgcttgttaaatttgagggcaatgatacatataattctatcttctttatagtgctgtttcagactctgctactcaattgtgttccctcccaaattcatatgttgaagtcctaaacctcagcaccttagaatatgaccttatttggagatcaggtctttaagttaaaaggaggacattgggaggggccctaatccaatcaatatgactggagtctttataaaaacaagaaatttggcctggggcggtgcctcatgcctgtaatcccagcactttgggagactgaggcaggtggatcacctgaggtcaggaatttgagaccagcctggccaacgtggtgaaaccccgtttctactaaaaatacaaaattagcctggcatggtggctgacgcctgttaaccccagctacttgggaagctgaggcagcagaatcacttgaacctgggaggcggaggttgcaatgagctgagatcgcgccactgtactccagcctgggcgacaagagtgaaattctgtctcaaaaaattaaaaaagcaaaaaaaaaaaaaaaaagaggaaatttgggggacagacttgcacacagggagaacaccatgtgaacatgaggctatccatctacaagccaaggacagacctgaaacagatccttcccccacaaccctcagaaggaaccaactgccaataactccattttgaatgtctggccttcacaactgtgagaccataaatttctgctaggtaggcaactcagtttgtagtaatttgttatggcagccatacgaactaatattgatgctaatttatcattttattaataaatgttgtaagttatacattttcatgccagcaacccctatctcccagatcttcctaactttaaatacttcagtgggttttctgtcaatgaacaatttgacatcagaaatttgggcaagagtcaggcataatggctcatgcctataatcccagtgatttggaaggccaaggtgggaggattgcttgagtccaggagtttgagactggcctgggcaacatagcgagatctcatctctacaagaaatttaaaaacttagcgggcatggtgccacatgcctgtagtcctagctatgcaggagggtgaagtgggaggattgctcgagcctgggagactacagcccgggagctatgatcaaccactgcactccatcctggacaacagaacgagaccatctctaagaaaaaaatattaagtctgtgaatgaatttatggttcctcaacagaaaatgaaacatcaagttatgaatgagttatgatatagttattttttattgtgtaagcccttattagttcctccctcatcccatcttaaaatattcaacaatagatagtggctcaaaaatttttttttaaaaaaacagactgccatgaaaaccaaatcttttcttcctgtaatagtggcttcctagtgttatttctcattaatgggagtatccgtggacttaactgtatattgcattttagttctggtcgtgtaataatttaatgacttcacacataaaaaactaatcttgtcttgagttttaaaaagttactagcacccatggttaaggaaggaaaactgtagctcacttcttcaatacatttgtttcttttcaattcatgaaatcagagaatatggaagaaacaggatgacagtcaccaagagtggttgaaactacaaactatcacgcaattgaaaataccacattaaagatatatttatatacagaaaatggagcaatgccaataaaattttataatttaaaaaagttacttgttaaaggcagatttcataagttgtgtttacaatcatccatttaatcatctccaaaaaaaggatgaatttattattttaaactaacattctgtaagttaaagagaataatcaagttgtctcatggactggaaggtgacttattaattccctttcatttccaaacctcatcaagcagtcactacatttatgaggcaagtcagctgaatgcttgaaatctagatgaattttaagatcttcaatttgtcctgttgaatattcacaatattgacataaataaatcccttcagataaatgtgaatttaaatgcttgcaatattctagcatacttgaaaagcctttcccacagtcatcacaaacatgaggaaaaatttttgtatgttcaatagcaacatgcctgttaacatttgtgtgaagtctactccgaaaaccacatacttgacatacaaagaagtttttacatttgtcaaaggtaattttgcttaagaggctatactgtccatgttcaccattgttatacttatcacttaactctattaatttacatgcatgctcatttaccacatggctatgcaagtcttctggatcattagtttcatgttcacagaactgacacaagtactgttcatcacagctgtgctcctggaaatgtaggtagagttcactgcttgaggagaactgtacatcacactgttcacaccaatagaggtgatcactaaaatgggtgtctgcaatgtgctggctgaggttctcaaaaattactgtcttataatcacagtatttacaaatgtagggatcctcttcatgcagtttggcatgttctatcagaagcatattggtagagaaactttccttgcatactcgacacacatttgaatcagtacgtttatgcttcaggatcatatgctgctttaagtcagaaaaatatttgctgttaaactcacaaagttcacatttatagaggccactgctattagctctcagtaaaggccatttctgctgggcagtcacattcaaagcttggctcttgtcaagaattttacaaagtttagctggcggttcttcatcagtttggtcttggagactctcagaggaattgttttctgtctctatatcataatcctcagaaatcgcatgcacttctacagcaattggaacatcttcagcagtgtgaacttctataggactctcctcttgggtttgctggttgactgattcaggtgagtcacactcttcatcacaaattacaatatcagcagatttttctgtagaaaaggcagtgtggtctagaattctaagtacaggactgggaaccaggtagttctgatttctgtttctggccttgattccatctgcaaattttggcaagtcatttgacgtctcggtatcagaatcatcatctttgttgtcaaaatattttaaatctggctgtctcatagaacagacactgtaacaatgatcagagaaaattccattgaatccatctgcaattctgcttattccagaggaatctgaataacgagaagggtgtagagtcttcctttttctttttttaggatactcattcatatcttttcaatttggtataattcttactactggagtgaggaaaaatgaattacaataagtttctgtagacagtaaaaaatgcctaacaatgtaaacaatcattccttgagtaaccatctcaattcacagtcagtcccccgaggccctcccggccggcccacgcagaggcggcggcggccgagagcgcaggcggaggggccgcgcggtccttcccgcggacgcacggcggcgggcagcgctgctccggccctagcgctcccggacgctgtgctgggccgacccctctccctccccgcgcgccccacgccctgagcgccaggcccctggcctaggctccgcggccgcactgccctggccgccacgctccgcgcctgcgccgcgcacctc

SEQ ID NO: 11215 - RNA, 4942 nt, Homo sapiens
  source 1..4942: mol_type = other RNA
ctgaatagctgggactacaggtgcccaccaccacgcccagctaatttttttttgtatttttagtagagacggggtttcactgttagccaggatggtctggatctcctgacctcgtgatctgcccatctcagccacccacaaagtgctgggattagaggcgtgggccaccacgcccagcctgcaatcttttcaattactaacacttgatccaaatgtaaagcagcaaatagattaaaagaaaacaaacaaaccaaggcattacttaaggtgtttttccaaaaatccaattcctggagctagatgtataaaaagcataaaaacaaaattatcaacaactaggttaattgttaggtgaagtagtcacaaaaaacatcccagggagaaaggttaggtttatgtaacatgatgtaatggaaacatcactagacagtaaaccagataacctggatcccactcccatgagacataactggttatatgtacttggcctcatagctatctacatttctatttctgcaaggaacttagaaaactggagggtttagaccagatgctttctaaggttatcttacaatttaaactgttacaattttaagtcttctgagaaacatttgttatcagccgtaacaggaatgttataattagatggaatgtgagttgctaggaacacaggtatgcacatacaacaaaatagtggggataaaaataataccttctaagaatacttgcagccaccattgtccaaacagactaaattcttgaagtgggaaaatcattggtcataaattgatcttccacttatatcaataaacctaaaaaataatgttagcagtgcttgttaaatttgagggcaatgatacatataattctatcttctttatagtgctgtttcagactctgctactcaattgtgttccctcccaaattcatatgttgaagtcctaaacctcagcaccttagaatatgaccttatttggagatcaggtctttaagttaaaaggaggacattgggaggggccctaatccaatcaatatgactggagtctttataaaaacaagaaatttggcctggggcggtgcctcatgcctgtaatcccagcactttgggagactgaggcaggtggatcacctgaggtcaggaatttgagaccagcctggccaacgtggtgaaaccccgtttctactaaaaatacaaaattagcctggcatggtggctgacgcctgttaaccccagctacttgggaagctgaggcagcagaatcacttgaacctgggaggcggaggttgcaatgagctgagatcgcgccactgtactccagcctgggcgacaagagtgaaattctgtctcaaaaaattaaaaaagcaaaaaaaaaaaaaaaaagaggaaatttgggggacagacttgcacacagggagaacaccatgtgaacatgaggctatccatctacaagccaaggacagacctgaaacagatccttcccccacaaccctcagaaggaaccaactgccaataactccattttgaatgtctggccttcacaactgtgagaccataaatttctgctaggtaggcaactcagtttgtagtaatttgttatggcagccatacgaactaatattgatgctaatttatcattttattaataaatgttgtaagttatacattttcatgccagcaacccctatctcccagatcttcctaactttaaatacttcagtgggttttctgtcaatgaacaatttgacatcagaaatttgggcaagagtcaggcataatggctcatgcctataatcccagtgatttggaaggccaaggtgggaggattgcttgagtccaggagtttgagactggcctgggcaacatagcgagatctcatctctacaagaaatttaaaaacttagcgggcatggtgccacatgcctgtagtcctagctatgcaggagggtgaagtgggaggattgctcgagcctgggagactacagcccgggagctatgatcaaccactgcactccatcctggacaacagaacgagaccatctctaagaaaaaaatattaagtctgtgaatgaatttatggttcctcaacagaaaatgaaacatcaagttatgaatgagttatgatatagttattttttattgtgtaagcccttattagttcctccctcatcccatcttaaaatattcaacaatagatagtggctcaaaaatttttttttaaaaaaacagactgccatgaaaaccaaatcttttcttcctgtaatagtggcttcctagtgttatttctcattaatgggagtatccgtggacttaactgtatattgcattttagttctggtcgtgtaataatttaatgacttcacacataaaaaactaatcttgtcttgagttttaaaaagttactagcacccatggttaaggaaggaaaactgtagctcacttcttcaatacatttgtttcttttcaattcatgaaatcagagaatatggaagaaacaggatgacagtcaccaagagtggttgaaactacaaactatcacgcaattgaaaataccacattaaagatatatttatatacagaaaatggagcaatgccaataaaattttataatttaaaaaagttacttgttaaaggcagatttcataagttgtgtttacaatcatccatttaatcatctccaaaaaaaggatgaatttattattttaaactaacattctgtaagttaaagagaataatcaagttgtctcatggactggaaggtgacttattaattccctttcatttccaaacctcatcaagcagtcactacatttatgaggcaagtcagctgaatgcttgaaatctagatgaattttaagatcttcaatttgtcctgttgaatattcacaatattgacataaataaatcccttcagataaatgtgaatttaaatgcttgcaatattctagcatacttgaaaagcctttcccacagtcatcacaaacatgaggaaaaatttttgtatgttcaatagcaacatgcctgttaacatttgtgtgaagtctactccgaaaaccacatacttgacatacaaagaagtttttacatttgtcaaaggtaattttgcttaagaggctatactgtccatgttcaccattgttatacttatcacttaactctattaatttacatgcatgctcatttaccacatggctatgcaagtcttctggatcattagtttcatgttcacagaactgacacaagtactgttcatcacagctgtgctcctggaaatgtaggtagagttcactgcttgaggagaactgtacatcacactgttcacaccaatagaggtgatcactaaaatgggtgtctgcaatgtgctggctgaggttctcaaaaattactgtcttataatcacagtatttacaaatgtagggatcctcttcatgcagtttggcatgttctatcagaagcatattggtagagaaactttccttgcatactcgacacacatttgaatcagtacgtttatgcttcaggatcatatgctgctttaagtcagaaaaatatttgctgttaaactcacaaagttcacatttatagaggccactgctattagctctcagtaaaggccatttctgctgggcagtcacattcaaagcttggctcttgtcaagaattttacaaagtttagctggcggttcttcatcagtttggtcttggagactctcagaggaattgttttctgtctctatatcataatcctcagaaatcgcatgcacttctacagcaattggaacatcttcagcagtgtgaacttctataggactctcctcttgggtttgctggttgactgattcaggtgagtcacactcttcatcacaaattacaatatcagcagatttttctgtagaaaaggcagtgtggtctagaattctaagtacaggactgggaaccaggtagttctgatttctgtttctggccttgattccatctgcaaattttggcaagtcatttgacgtctcggtatcagaatcatcatctttgttgtcaaaatattttaaatctggctgtctcatagaacagacactgtaacaatgatcagagaaaattccattgaatccatctgcaattctgcttattccagaggaatctgaataacgagaagggtgtagagtcttcctttttctttttttaggatactcattcatatcttttcaatttggtataattcttactactggagtgaggaaaaatgaattacaataagtttctgtagacagtaaaaaatgcctcgccgggtgcagtggttcacgcctgtaatcccagcactttgggaggccgaggcgaacagatcacctgaggtcgggaattcaagactagcctgaccaacatggggaaaccccgtctcgactgaaaatacaaaattagccgggcgtggtggcacatgcctgtaatctgagctactcgggaggctgaggcatgagaatcgcttgaatccgggaggcggaggttgtggtgacccgagatcacatcattgtcctccagcctgggtaacaggagtgaaactcgtcacacgagtgaggcgactctcaggctggaggctttgggcgccagcatcgacgcctgctctccgcggctacaactcgttgcgcgagcccggggattcgccgccggaggtcacgaagccgccgggcagggccgcagcgccagcgaggacccaggatcgtcccgagcccggacgcagccagacaaatgcccgtcggaggcgcagggcagaagtccctgggacttagccgcctccaccccggcgccacgcaccagcttcgcccgggcccagaagccggcgccaaggagacttccaagccccgacaccaaaggttccgtaaagacaacggcagcagggggccgaggggagcccggccaaggcgtcctgcgcagggggtggaactgccttcggga

SEQ ID NO: 11216 - RNA, 4695 nt, Homo sapiens
  source 1..4695: mol_type = other RNA
ctgaatagctgggactacaggtgcccaccaccacgcccagctaatttttttttgtatttttagtagagacggggtttcactgttagccaggatggtctggatctcctgacctcgtgatctgcccatctcagccacccacaaagtgctgggattagaggcgtgggccaccacgcccagcctgcaatcttttcaattactaacacttgatccaaatgtaaagcagcaaatagattaaaagaaaacaaacaaaccaaggcattacttaaggtgtttttccaaaaatccaattcctggagctagatgtataaaaagcataaaaacaaaattatcaacaactaggttaattgttaggtgaagtagtcacaaaaaacatcccagggagaaaggttaggtttatgtaacatgatgtaatggaaacatcactagacagtaaaccagataacctggatcccactcccatgagacataactggttatatgtacttggcctcatagctatctacatttctatttctgcaaggaacttagaaaactggagggtttagaccagatgctttctaaggttatcttacaatttaaactgttacaattttaagtcttctgagaaacatttgttatcagccgtaacaggaatgttataattagatggaatgtgagttgctaggaacacaggtatgcacatacaacaaaatagtggggataaaaataataccttctaagaatacttgcagccaccattgtccaaacagactaaattcttgaagtgggaaaatcattggtcataaattgatcttccacttatatcaataaacctaaaaaataatgttagcagtgcttgttaaatttgagggcaatgatacatataattctatcttctttatagtgctgtttcagactctgctactcaattgtgttccctcccaaattcatatgttgaagtcctaaacctcagcaccttagaatatgaccttatttggagatcaggtctttaagttaaaaggaggacattgggaggggccctaatccaatcaatatgactggagtctttataaaaacaagaaatttggcctggggcggtgcctcatgcctgtaatcccagcactttgggagactgaggcaggtggatcacctgaggtcaggaatttgagaccagcctggccaacgtggtgaaaccccgtttctactaaaaatacaaaattagcctggcatggtggctgacgcctgttaaccccagctacttgggaagctgaggcagcagaatcacttgaacctgggaggcggaggttgcaatgagctgagatcgcgccactgtactccagcctgggcgacaagagtgaaattctgtctcaaaaaattaaaaaagcaaaaaaaaaaaaaaaaagaggaaatttgggggacagacttgcacacagggagaacaccatgtgaacatgaggctatccatctacaagccaaggacagacctgaaacagatccttcccccacaaccctcagaaggaaccaactgccaataactccattttgaatgtctggccttcacaactgtgagaccataaatttctgctaggtaggcaactcagtttgtagtaatttgttatggcagccatacgaactaatattgatgctaatttatcattttattaataaatgttgtaagttatacattttcatgccagcaacccctatctcccagatcttcctaactttaaatacttcagtgggttttctgtcaatgaacaatttgacatcagaaatttgggcaagagtcaggcataatggctcatgcctataatcccagtgatttggaaggccaaggtgggaggattgcttgagtccaggagtttgagactggcctgggcaacatagcgagatctcatctctacaagaaatttaaaaacttagcgggcatggtgccacatgcctgtagtcctagctatgcaggagggtgaagtgggaggattgctcgagcctgggagactacagcccgggagctatgatcaaccactgcactccatcctggacaacagaacgagaccatctctaagaaaaaaatattaagtctgtgaatgaatttatggttcctcaacagaaaatgaaacatcaagttatgaatgagttatgatatagttattttttattgtgtaagcccttattagttcctccctcatcccatcttaaaatattcaacaatagatagtggctcaaaaatttttttttaaaaaaacagactgccatgaaaaccaaatcttttcttcctgtaatagtggcttcctagtgttatttctcattaatgggagtatccgtggacttaactgtatattgcattttagttctggtcgtgtaataatttaatgacttcacacataaaaaactaatcttgtcttgagttttaaaaagttactagcacccatggttaaggaaggaaaactgtagctcacttcttcaatacatttgtttcttttcaattcatgaaatcagagaatatggaagaaacaggatgacagtcaccaagagtggttgaaactacaaactatcacgcaattgaaaataccacattaaagatatatttatatacagaaaatggagcaatgccaataaaattttataatttaaaaaagttacttgttaaaggcagatttcataagttgtgtttacaatcatccatttaatcatctccaaaaaaaggatgaatttattattttaaactaacattctgtaagttaaagagaataatcaagttgtctcatggactggaaggtgacttattaattccctttcatttccaaacctcatcaagcagtcactacatttatgaggcaagtcagctgaatgcttgaaatctagatgaattttaagatcttcaatttgtcctgttgaatattcacaatattgacataaataaatcccttcagataaatgtgaatttaaatgcttgcaatattctagcatacttgaaaagcctttcccacagtcatcacaaacatgaggaaaaatttttgtatgttcaatagcaacatgcctgttaacatttgtgtgaagtctactccgaaaaccacatacttgacatacaaagaagtttttacatttgtcaaaggtaattttgcttaagaggctatactgtccatgttcaccattgttatacttatcacttaactctattaatttacatgcatgctcatttaccacatggctatgcaagtcttctggatcattagtttcatgttcacagaactgacacaagtactgttcatcacagctgtgctcctggaaatgtaggtagagttcactgcttgaggagaactgtacatcacactgttcacaccaatagaggtgatcactaaaatgggtgtctgcaatgtgctggctgaggttctcaaaaattactgtcttataatcacagtatttacaaatgtagggatcctcttcatgcagtttggcatgttctatcagaagcatattggtagagaaactttccttgcatactcgacacacatttgaatcagtacgtttatgcttcaggatcatatgctgctttaagtcagaaaaatatttgctgttaaactcacaaagttcacatttatagaggccactgctattagctctcagtaaaggccatttctgctgggcagtcacattcaaagcttggctcttgtcaagaattttacaaagtttagctggcggttcttcatcagtttggtcttggagactctcagaggaattgttttctgtctctatatcataatcctcagaaatcgcatgcacttctacagcaattggaacatcttcagcagtgtgaacttctataggactctcctcttgggtttgctggttgactgattcaggtgagtcacactcttcatcacaaattacaatatcagcagatttttctgtagaaaaggcagtgtggtctagaattctaagtacaggactgggaaccaggtagttctgatttctgtttctggccttgattccatctgcaaattttggcaagtcatttgacgtctcggtatcagaatcatcatctttgttgtcaaaatattttaaatctggctgtctcatagaacagacactgtaacaatgatcagagaaaattccattgaatccatctgcaattctgcttattccagaggaatctgaataacgagaagggtgtagagtcttcctttttctttttttaggatactcattcatatcttttcaatttggtataattcttactactggagtgaggaaaaatgaattacaataagtttctgtagacagtaaaaaatgcctcgccgggtgcagtggttcacgcctgtaatcccagcactttgggaggccgaggcgaacagatcacctgaggtcgggaattcaagactagcctgaccaacatggggaaaccccgtctcgactgaaaatacaaaattagccgggcgtggtggcacatgcctgtaatctgagctactcgggaggctgaggcatgagaatcgcttgaatccgggaggcggaggttgtggtgacccgagatcacatcattgtcctccagcctgggtaacaggagtgaaactctgtcagcttcgcccgggcccagaagccggcgccaaggagacttccaagccccgacaccaaaggttccgtaaagacaacggcagcagggggccgaggggagcccggccaaggcgtcctgcgcagggggtggaactgccttcggga

SEQ ID NO: 11217 - RNA, 4815 nt, Homo sapiens
  source 1..4815: mol_type = other RNA
ctgaatagctgggactacaggtgcccaccaccacgcccagctaatttttttttgtatttttagtagagacggggtttcactgttagccaggatggtctggatctcctgacctcgtgatctgcccatctcagccacccacaaagtgctgggattagaggcgtgggccaccacgcccagcctgcaatcttttcaattactaacacttgatccaaatgtaaagcagcaaatagattaaaagaaaacaaacaaaccaaggcattacttaaggtgtttttccaaaaatccaattcctggagctagatgtataaaaagcataaaaacaaaattatcaacaactaggttaattgttaggtgaagtagtcacaaaaaacatcccagggagaaaggttaggtttatgtaacatgatgtaatggaaacatcactagacagtaaaccagataacctggatcccactcccatgagacataactggttatatgtacttggcctcatagctatctacatttctatttctgcaaggaacttagaaaactggagggtttagaccagatgctttctaaggttatcttacaatttaaactgttacaattttaagtcttctgagaaacatttgttatcagccgtaacaggaatgttataattagatggaatgtgagttgctaggaacacaggtatgcacatacaacaaaatagtggggataaaaataataccttctaagaatacttgcagccaccattgtccaaacagactaaattcttgaagtgggaaaatcattggtcataaattgatcttccacttatatcaataaacctaaaaaataatgttagcagtgcttgttaaatttgagggcaatgatacatataattctatcttctttatagtgctgtttcagactctgctactcaattgtgttccctcccaaattcatatgttgaagtcctaaacctcagcaccttagaatatgaccttatttggagatcaggtctttaagttaaaaggaggacattgggaggggccctaatccaatcaatatgactggagtctttataaaaacaagaaatttggcctggggcggtgcctcatgcctgtaatcccagcactttgggagactgaggcaggtggatcacctgaggtcaggaatttgagaccagcctggccaacgtggtgaaaccccgtttctactaaaaatacaaaattagcctggcatggtggctgacgcctgttaaccccagctacttgggaagctgaggcagcagaatcacttgaacctgggaggcggaggttgcaatgagctgagatcgcgccactgtactccagcctgggcgacaagagtgaaattctgtctcaaaaaattaaaaaagcaaaaaaaaaaaaaaaaagaggaaatttgggggacagacttgcacacagggagaacaccatgtgaacatgaggctatccatctacaagccaaggacagacctgaaacagatccttcccccacaaccctcagaaggaaccaactgccaataactccattttgaatgtctggccttcacaactgtgagaccataaatttctgctaggtaggcaactcagtttgtagtaatttgttatggcagccatacgaactaatattgatgctaatttatcattttattaataaatgttgtaagttatacattttcatgccagcaacccctatctcccagatcttcctaactttaaatacttcagtgggttttctgtcaatgaacaatttgacatcagaaatttgggcaagagtcaggcataatggctcatgcctataatcccagtgatttggaaggccaaggtgggaggattgcttgagtccaggagtttgagactggcctgggcaacatagcgagatctcatctctacaagaaatttaaaaacttagcgggcatggtgccacatgcctgtagtcctagctatgcaggagggtgaagtgggaggattgctcgagcctgggagactacagcccgggagctatgatcaaccactgcactccatcctggacaacagaacgagaccatctctaagaaaaaaatattaagtctgtgaatgaatttatggttcctcaacagaaaatgaaacatcaagttatgaatgagttatgatatagttattttttattgtgtaagcccttattagttcctccctcatcccatcttaaaatattcaacaatagatagtggctcaaaaatttttttttaaaaaaacagactgccatgaaaaccaaatcttttcttcctgtaatagtggcttcctagtgttatttctcattaatgggagtatccgtggacttaactgtatattgcattttagttctggtcgtgtaataatttaatgacttcacacataaaaaactaatcttgtcttgagttttaaaaagttactagcacccatggttaaggaaggaaaactgtagctcacttcttcaatacatttgtttcttttcaattcatgaaatcagagaatatggaagaaacaggatgacagtcaccaagagtggttgaaactacaaactatcacgcaattgaaaataccacattaaagatatatttatatacagaaaatggagcaatgccaataaaattttataatttaaaaaagttacttgttaaaggcagatttcataagttgtgtttacaatcatccatttaatcatctccaaaaaaaggatgaatttattattttaaactaacattctgtaagttaaagagaataatcaagttgtctcatggactggaaggtgacttattaattccctttcatttccaaacctcatcaagcagtcactacatttatgaggcaagtcagctgaatgcttgaaatctagatgaattttaagatcttcaatttgtcctgttgaatattcacaatattgacataaataaatcccttcagataaatgtgaatttaaatgcttgcaatattctagcatacttgaaaagcctttcccacagtcatcacaaacatgaggaaaaatttttgtatgttcaatagcaacatgcctgttaacatttgtgtgaagtctactccgaaaaccacatacttgacatacaaagaagtttttacatttgtcaaaggtaattttgcttaagaggctatactgtccatgttcaccattgttatacttatcacttaactctattaatttacatgcatgctcatttaccacatggctatgcaagtcttctggatcattagtttcatgttcacagaactgacacaagtactgttcatcacagctgtgctcctggaaatgtaggtagagttcactgcttgaggagaactgtacatcacactgttcacaccaatagaggtgatcactaaaatgggtgtctgcaatgtgctggctgaggttctcaaaaattactgtcttataatcacagtatttacaaatgtagggatcctcttcatgcagtttggcatgttctatcagaagcatattggtagagaaactttccttgcatactcgacacacatttgaatcagtacgtttatgcttcaggatcatatgctgctttaagtcagaaaaatatttgctgttaaactcacaaagttcacatttatagaggccactgctattagctctcagtaaaggccatttctgctgggcagtcacattcaaagcttggctcttgtcaagaattttacaaagtttagctggcggttcttcatcagtttggtcttggagactctcagaggaattgttttctgtctctatatcataatcctcagaaatcgcatgcacttctacagcaattggaacatcttcagcagtgtgaacttctataggactctcctcttgggtttgctggttgactgattcaggtgagtcacactcttcatcacaaattacaatatcagcagatttttctgtagaaaaggcagtgtggtctagaattctaagtacaggactgggaaccaggtagttctgatttctgtttctggccttgattccatctgcaaattttggcaagtcatttgacgtctcggtatcagaatcatcatctttgttgtcaaaatattttaaatctggctgtctcatagaacagacactgtaacaatgatcagagaaaattccattgaatccatctgcaattctgcttattccagaggaatctgaataacgagaagggtgtagagtcttcctttttctttttttaggatactcattcatatcttttcaatttggtataattcttactactggagtgaggaaaaatgaattacaataagtttctgtagacagtaaaaaatgcctcgccgggtgcagtggttcacgcctgtaatcccagcactttgggaggccgaggcgaacagatcacctgaggtcgggaattcaagactagcctgaccaacatggggaaaccccgtctcgactgaaaatacaaaattagccgggcgtggtggcacatgcctgtaatctgagctactcgggaggctgaggcatgagaatcgcttgaatccgggaggcggaggttgtggtgacccgagatcacatcattgtcctccagcctgggtaacaggagtgaaactctgtcagtcagtcccccgaggccctcccggccggcccacgcagaggcggcggcggccgagagcgcaggcggaggggccgcgcggtccttcccgcggacgcacggcggcgggcagcgctgctccggccctagcgctcccggacgctgtgctgggccgacccctctccctccccgcgcgccccacgccctgagcgccaggcccctggcctaggctccgcggccgcactgccctggccgccacgctccgcgcctgcgccgcgcacctc

SEQ ID NO: 11218 - RNA, 4639 nt, Homo sapiens
  source 1..4639: mol_type = other RNA
ctgaatagctgggactacaggtgcccaccaccacgcccagctaatttttttttgtatttttagtagagacggggtttcactgttagccaggatggtctggatctcctgacctcgtgatctgcccatctcagccacccacaaagtgctgggattagaggcgtgggccaccacgcccagcctgcaatcttttcaattactaacacttgatccaaatgtaaagcagcaaatagattaaaagaaaacaaacaaaccaaggcattacttaaggtgtttttccaaaaatccaattcctggagctagatgtataaaaagcataaaaacaaaattatcaacaactaggttaattgttaggtgaagtagtcacaaaaaacatcccagggagaaaggttaggtttatgtaacatgatgtaatggaaacatcactagacagtaaaccagataacctggatcccactcccatgagacataactggttatatgtacttggcctcatagctatctacatttctatttctgcaaggaacttagaaaactggagggtttagaccagatgctttctaaggttatcttacaatttaaactgttacaattttaagtcttctgagaaacatttgttatcagccgtaacaggaatgttataattagatggaatgtgagttgctaggaacacaggtatgcacatacaacaaaatagtggggataaaaataataccttctaagaatacttgcagccaccattgtccaaacagactaaattcttgaagtgggaaaatcattggtcataaattgatcttccacttatatcaataaacctaaaaaataatgttagcagtgcttgttaaatttgagggcaatgatacatataattctatcttctttatagtgctgtttcagactctgctactcaattgtgttccctcccaaattcatatgttgaagtcctaaacctcagcaccttagaatatgaccttatttggagatcaggtctttaagttaaaaggaggacattgggaggggccctaatccaatcaatatgactggagtctttataaaaacaagaaatttggcctggggcggtgcctcatgcctgtaatcccagcactttgggagactgaggcaggtggatcacctgaggtcaggaatttgagaccagcctggccaacgtggtgaaaccccgtttctactaaaaatacaaaattagcctggcatggtggctgacgcctgttaaccccagctacttgggaagctgaggcagcagaatcacttgaacctgggaggcggaggttgcaatgagctgagatcgcgccactgtactccagcctgggcgacaagagtgaaattctgtctcaaaaaattaaaaaagcaaaaaaaaaaaaaaaaagaggaaatttgggggacagacttgcacacagggagaacaccatgtgaacatgaggctatccatctacaagccaaggacagacctgaaacagatccttcccccacaaccctcagaaggaaccaactgccaataactccattttgaatgtctggccttcacaactgtgagaccataaatttctgctaggtaggcaactcagtttgtagtaatttgttatggcagccatacgaactaatattgatgctaatttatcattttattaataaatgttgtaagttatacattttcatgccagcaacccctatctcccagatcttcctaactttaaatacttcagtgggttttctgtcaatgaacaatttgacatcagaaatttgggcaagagtcaggcataatggctcatgcctataatcccagtgatttggaaggccaaggtgggaggattgcttgagtccaggagtttgagactggcctgggcaacatagcgagatctcatctctacaagaaatttaaaaacttagcgggcatggtgccacatgcctgtagtcctagctatgcaggagggtgaagtgggaggattgctcgagcctgggagactacagcccgggagctatgatcaaccactgcactccatcctggacaacagaacgagaccatctctaagaaaaaaatattaagtctgtgaatgaatttatggttcctcaacagaaaatgaaacatcaagttatgaatgagttatgatatagttattttttattgtgtaagcccttattagttcctccctcatcccatcttaaaatattcaacaatagatagtggctcaaaaatttttttttaaaaaaacagactgccatgaaaaccaaatcttttcttcctgtaatagtggcttcctagtgttatttctcattaatgggagtatccgtggacttaactgtatattgcattttagttctggtcgtgtaataatttaatgacttcacacataaaaaactaatcttgtcttgagttttaaaaagttactagcacccatggttaaggaaggaaaactgtagctcacttcttcaatacatttgtttcttttcaattcatgaaatcagagaatatggaagaaacaggatgacagtcaccaagagtggttgaaactacaaactatcacgcaattgaaaataccacattaaagatatatttatatacagaaaatggagcaatgccaataaaattttataatttaaaaaagttacttgttaaaggcagatttcataagttgtgtttacaatcatccatttaatcatctccaaaaaaaggatgaatttattattttaaactaacattctgtaagttaaagagaataatcaagttgtctcatggactggaaggtgacttattaattccctttcatttccaaacctcatcaagcagtcactacatttatgaggcaagtcagctgaatgcttgaaatctagatgaattttaagatcttcaatttgtcctgttgaatattcacaatattgacataaataaatcccttcagataaatgtgaatttaaatgcttgcaatattctagcatacttgaaaagcctttcccacagtcatcacaaacatgaggaaaaatttttgtatgttcaatagcaacatgcctgttaacatttgtgtgaagtctactccgaaaaccacatacttgacatacaaagaagtttttacatttgtcaaaggtaattttgcttaagaggctatactgtccatgttcaccattgttatacttatcacttaactctattaatttacatgcatgctcatttaccacatggctatgcaagtcttctggatcattagtttcatgttcacagaactgacacaagtactgttcatcacagctgtgctcctggaaatgtaggtagagttcactgcttgaggagaactgtacatcacactgttcacaccaatagaggtgatcactaaaatgggtgtctgcaatgtgctggctgaggttctcaaaaattactgtcttataatcacagtatttacaaatgtagggatcctcttcatgcagtttggcatgttctatcagaagcatattggtagagaaactttccttgcatactcgacacacatttgaatcagtacgtttatgcttcaggatcatatgctgctttaagtcagaaaaatatttgctgttaaactcacaaagttcacatttatagaggccactgctattagctctcagtaaaggccatttctgctgggcagtcacattcaaagcttggctcttgtcaagaattttacaaagtttagctggcggttcttcatcagtttggtcttggagactctcagaggaattgttttctgtctctatatcataatcctcagaaatcgcatgcacttctacagcaattggaacatcttcagcagtgtgaacttctataggactctcctcttgggtttgctggttgactgattcaggtgagtcacactcttcatcacaaattacaatatcagcagatttttctgtagaaaaggcagtgtggtctagaattctaagtacaggactgggaaccaggtagttctgatttctgtttctggccttgattccatctgcaaattttggcaagtcatttgacgtctcggtatcagaatcatcatctttgttgtcaaaatattttaaatctggctgtctcatagaacagacactgtaacaatgatcagagaaaattccattgaatccatctgcaattctgcttattccagaggaatctgaataacgagaagggtgtagagtcttcctttttctttttttaggatactcattcatatcttttcaatttggtataattcttactactggagtgaggaaaaatgaattacaataagtttctgtagacagtaaaaaatgcctcgccgggtgcagtggttcacgcctgtaatcccagcactttgggaggccgaggcgaacagatcacctgaggtcgggaattcaagactagcctgaccaacatggggaaaccccgtctcgactgaaaatacaaaattagccgggcgtggtggcacatgcctgtaatctgagctactcgggaggctgaggcatgagaatcgcttgaatccgggaggcggaggttgtggtgacccgagatcacatcattgtcctccagcctgggtaacaggagtgaaactctgtcgcacacgcggcctgggagggaccaccggcccgcagccccgggggaggcccagcggcccgcgccccctgccggaggccttgcgcc

SEQ ID NO: 11219 - RNA, 4946 nt, Homo sapiens
  source 1..4946: mol_type = other RNA
ctgaatagctgggactacaggtgcccaccaccacgcccagctaatttttttttgtatttttagtagagacggggtttcactgttagccaggatggtctggatctcctgacctcgtgatctgcccatctcagccacccacaaagtgctgggattagaggcgtgggccaccacgcccagcctgcaatcttttcaattactaacacttgatccaaatgtaaagcagcaaatagattaaaagaaaacaaacaaaccaaggcattacttaaggtgtttttccaaaaatccaattcctggagctagatgtataaaaagcataaaaacaaaattatcaacaactaggttaattgttaggtgaagtagtcacaaaaaacatcccagggagaaaggttaggtttatgtaacatgatgtaatggaaacatcactagacagtaaaccagataacctggatcccactcccatgagacataactggttatatgtacttggcctcatagctatctacatttctatttctgcaaggaacttagaaaactggagggtttagaccagatgctttctaaggttatcttacaatttaaactgttacaattttaagtcttctgagaaacatttgttatcagccgtaacaggaatgttataattagatggaatgtgagttgctaggaacacaggtatgcacatacaacaaaatagtggggataaaaataataccttctaagaatacttgcagccaccattgtccaaacagactaaattcttgaagtgggaaaatcattggtcataaattgatcttccacttatatcaataaacctaaaaaataatgttagcagtgcttgttaaatttgagggcaatgatacatataattctatcttctttatagtgctgtttcagactctgctactcaattgtgttccctcccaaattcatatgttgaagtcctaaacctcagcaccttagaatatgaccttatttggagatcaggtctttaagttaaaaggaggacattgggaggggccctaatccaatcaatatgactggagtctttataaaaacaagaaatttggcctggggcggtgcctcatgcctgtaatcccagcactttgggagactgaggcaggtggatcacctgaggtcaggaatttgagaccagcctggccaacgtggtgaaaccccgtttctactaaaaatacaaaattagcctggcatggtggctgacgcctgttaaccccagctacttgggaagctgaggcagcagaatcacttgaacctgggaggcggaggttgcaatgagctgagatcgcgccactgtactccagcctgggcgacaagagtgaaattctgtctcaaaaaattaaaaaagcaaaaaaaaaaaaaaaaagaggaaatttgggggacagacttgcacacagggagaacaccatgtgaacatgaggctatccatctacaagccaaggacagacctgaaacagatccttcccccacaaccctcagaaggaaccaactgccaataactccattttgaatgtctggccttcacaactgtgagaccataaatttctgctaggtaggcaactcagtttgtagtaatttgttatggcagccatacgaactaatattgatgctaatttatcattttattaataaatgttgtaagttatacattttcatgccagcaacccctatctcccagatcttcctaactttaaatacttcagtgggttttctgtcaatgaacaatttgacatcagaaatttgggcaagagtcaggcataatggctcatgcctataatcccagtgatttggaaggccaaggtgggaggattgcttgagtccaggagtttgagactggcctgggcaacatagcgagatctcatctctacaagaaatttaaaaacttagcgggcatggtgccacatgcctgtagtcctagctatgcaggagggtgaagtgggaggattgctcgagcctgggagactacagcccgggagctatgatcaaccactgcactccatcctggacaacagaacgagaccatctctaagaaaaaaatattaagtctgtgaatgaatttatggttcctcaacagaaaatgaaacatcaagttatgaatgagttatgatatagttattttttattgtgtaagcccttattagttcctccctcatcccatcttaaaatattcaacaatagatagtggctcaaaaatttttttttaaaaaaacagactgccatgaaaaccaaatcttttcttcctgtaatagtggcttcctagtgttatttctcattaatgggagtatccgtggacttaactgtatattgcattttagttctggtcgtgtaataatttaatgacttcacacataaaaaactaatcttgtcttgagttttaaaaagttactagcacccatggttaaggaaggaaaactgtagctcacttcttcaatacatttgtttcttttcaattcatgaaatcagagaatatggaagaaacaggatgacagtcaccaagagtggttgaaactacaaactatcacgcaattgaaaataccacattaaagatatatttatatacagaaaatggagcaatgccaataaaattttataatttaaaaaagttacttgttaaaggcagatttcataagttgtgtttacaatcatccatttaatcatctccaaaaaaaggatgaatttattattttaaactaacattctgtaagttaaagagaataatcaagttgtctcatggactggaaggtgacttattaattccctttcatttccaaacctcatcaagcagtcactacatttatgaggcaagtcagctgaatgcttgaaatctagatgaattttaagatcttcaatttgtcctgttgaatattcacaatattgacataaataaatcccttcagataaatgtgaatttaaatgcttgcaatattctagcatacttgaaaagcctttcccacagtcatcacaaacatgaggaaaaatttttgtatgttcaatagcaacatgcctgttaacatttgtgtgaagtctactccgaaaaccacatacttgacatacaaagaagtttttacatttgtcaaaggtaattttgcttaagaggctatactgtccatgttcaccattgttatacttatcacttaactctattaatttacatgcatgctcatttaccacatggctatgcaagtcttctggatcattagtttcatgttcacagaactgacacaagtactgttcatcacagctgtgctcctggaaatgtaggtagagttcactgcttgaggagaactgtacatcacactgttcacaccaatagaggtgatcactaaaatgggtgtctgcaatgtgctggctgaggttctcaaaaattactgtcttataatcacagtatttacaaatgtagggatcctcttcatgcagtttggcatgttctatcagaagcatattggtagagaaactttccttgcatactcgacacacatttgaatcagtacgtttatgcttcaggatcatatgctgctttaagtcagaaaaatatttgctgttaaactcacaaagttcacatttatagaggccactgctattagctctcagtaaaggccatttctgctgggcagtcacattcaaagcttggctcttgtcaagaattttacaaagtttagctggcggttcttcatcagtttggtcttggagactctcagaggaattgttttctgtctctatatcataatcctcagaaatcgcatgcacttctacagcaattggaacatcttcagcagtgtgaacttctataggactctcctcttgggtttgctggttgactgattcaggtgagtcacactcttcatcacaaattacaatatcagcagatttttctgtagaaaaggcagtgtggtctagaattctaagtacaggactgggaaccaggtagttctgatttctgtttctggccttgattccatctgcaaattttggcaagtcatttgacgtctcggtatcagaatcatcatctttgttgtcaaaatattttaaatctggctgtctcatagaacagacactgtaacaatgatcagagaaaattccattgaatccatctgcaattctgcttattccagaggaatctgaataacgagaagggtgtagagtcttcctttttctttttttaggatactcattcatatcttttcaatttggtataattcttactactggagtgaggaaaaatgaattacaataagtttctgtagacagtaaaaaatgcctcgccgggtgcagtggttcacgcctgtaatcccagcactttgggaggccgaggcgaacagatcacctgaggtcgggaattcaagactagcctgaccaacatggggaaaccccgtctcgactgaaaatacaaaattagccgggcgtggtggcacatgcctgtaatctgagctactcgggaggctgaggcatgagaatcgcttgaatccgggaggcggaggttgtggtgacccgagatcacatcattgtcctccagcctgggtaacaggagtgaaactctgtcgtcacacgagtgaggcgactctcaggctggaggctttgggcgccagcatcgacgcctgctctccgcggctacaactcgttgcgcgagcccggggattcgccgccggaggtcacgaagccgccgggcagggccgcagcgccagcgaggacccaggatcgtcccgagcccggacgcagccagacaaatgcccgtcggaggcgcagggcagaagtccctgggacttagccgcctccaccccggcgccacgcaccagcttcgcccgggcccagaagccggcgccaaggagacttccaagccccgacaccaaaggttccgtaaagacaacggcagcagggggccgaggggagcccggccaaggcgtcctgcgcagggggtggaactgccttcggga

SEQ ID NO: 11220 - RNA, 4868 nt, Homo sapiens
  source 1..4868: mol_type = other RNA
ctgaatagctgggactacaggtgcccaccaccacgcccagctaatttttttttgtatttttagtagagacggggtttcactgttagccaggatggtctggatctcctgacctcgtgatctgcccatctcagccacccacaaagtgctgggattagaggcgtgggccaccacgcccagcctgcaatcttttcaattactaacacttgatccaaatgtaaagcagcaaatagattaaaagaaaacaaacaaaccaaggcattacttaaggtgtttttccaaaaatccaattcctggagctagatgtataaaaagcataaaaacaaaattatcaacaactaggttaattgttaggtgaagtagtcacaaaaaacatcccagggagaaaggttaggtttatgtaacatgatgtaatggaaacatcactagacagtaaaccagataacctggatcccactcccatgagacataactggttatatgtacttggcctcatagctatctacatttctatttctgcaaggaacttagaaaactggagggtttagaccagatgctttctaaggttatcttacaatttaaactgttacaattttaagtcttctgagaaacatttgttatcagccgtaacaggaatgttataattagatggaatgtgagttgctaggaacacaggtatgcacatacaacaaaatagtggggataaaaataataccttctaagaatacttgcagccaccattgtccaaacagactaaattcttgaagtgggaaaatcattggtcataaattgatcttccacttatatcaataaacctaaaaaataatgttagcagtgcttgttaaatttgagggcaatgatacatataattctatcttctttatagtgctgtttcagactctgctactcaattgtgttccctcccaaattcatatgttgaagtcctaaacctcagcaccttagaatatgaccttatttggagatcaggtctttaagttaaaaggaggacattgggaggggccctaatccaatcaatatgactggagtctttataaaaacaagaaatttggcctggggcggtgcctcatgcctgtaatcccagcactttgggagactgaggcaggtggatcacctgaggtcaggaatttgagaccagcctggccaacgtggtgaaaccccgtttctactaaaaatacaaaattagcctggcatggtggctgacgcctgttaaccccagctacttgggaagctgaggcagcagaatcacttgaacctgggaggcggaggttgcaatgagctgagatcgcgccactgtactccagcctgggcgacaagagtgaaattctgtctcaaaaaattaaaaaagcaaaaaaaaaaaaaaaaagaggaaatttgggggacagacttgcacacagggagaacaccatgtgaacatgaggctatccatctacaagccaaggacagacctgaaacagatccttcccccacaaccctcagaaggaaccaactgccaataactccattttgaatgtctggccttcacaactgtgagaccataaatttctgctaggtaggcaactcagtttgtagtaatttgttatggcagccatacgaactaatattgatgctaatttatcattttattaataaatgttgtaagttatacattttcatgccagcaacccctatctcccagatcttcctaactttaaatacttcagtgggttttctgtcaatgaacaatttgacatcagaaatttgggcaagagtcaggcataatggctcatgcctataatcccagtgatttggaaggccaaggtgggaggattgcttgagtccaggagtttgagactggcctgggcaacatagcgagatctcatctctacaagaaatttaaaaacttagcgggcatggtgccacatgcctgtagtcctagctatgcaggagggtgaagtgggaggattgctcgagcctgggagactacagcccgggagctatgatcaaccactgcactccatcctggacaacagaacgagaccatctctaagaaaaaaatattaagtctgtgaatgaatttatggttcctcaacagaaaatgaaacatcaagttatgaatgagttatgatatagttattttttattgtgtaagcccttattagttcctccctcatcccatcttaaaatattcaacaatagatagtggctcaaaaatttttttttaaaaaaacagactgccatgaaaaccaaatcttttcttcctgtaatagtggcttcctagtgttatttctcattaatgggagtatccgtggacttaactgtatattgcattttagttctggtcgtgtaataatttaatgacttcacacataaaaaactaatcttgtcttgagttttaaaaagttactagcacccatggttaaggaaggaaaactgtagctcacttcttcaatacatttgtttcttttcaattcatgaaatcagagaatatggaagaaacaggatgacagtcaccaagagtggttgaaactacaaactatcacgcaattgaaaataccacattaaagatatatttatatacagaaaatggagcaatgccaataaaattttataatttaaaaaagttacttgttaaaggcagatttcataagttgtgtttacaatcatccatttaatcatctccaaaaaaaggatgaatttattattttaaactaacattctgtaagttaaagagaataatcaagttgtctcatggactggaaggtgacttattaattccctttcatttccaaacctcatcaagcagtcactacatttatgaggcaagtcagctgaatgcttgaaatctagatgaattttaagatcttcaatttgtcctgttgaatattcacaatattgacataaataaatcccttcagataaatgtgaatttaaatgcttgcaatattctagcatacttgaaaagcctttcccacagtcatcacaaacatgaggaaaaatttttgtatgttcaatagcaacatgcctgttaacatttgtgtgaagtctactccgaaaaccacatacttgacatacaaagaagtttttacatttgtcaaaggtaattttgcttaagaggctatactgtccatgttcaccattgttatacttatcacttaactctattaatttacatgcatgctcatttaccacatggctatgcaagtcttctggatcattagtttcatgttcacagaactgacacaagtactgttcatcacagctgtgctcctggaaatgtaggtagagttcactgcttgaggagaactgtacatcacactgttcacaccaatagaggtgatcactaaaatgggtgtctgcaatgtgctggctgaggttctcaaaaattactgtcttataatcacagtatttacaaatgtagggatcctcttcatgcagtttggcatgttctatcagaagcatattggtagagaaactttccttgcatactcgacacacatttgaatcagtacgtttatgcttcaggatcatatgctgctttaagtcagaaaaatatttgctgttaaactcacaaagttcacatttatagaggccactgctattagctctcagtaaaggccatttctgctgggcagtcacattcaaagcttggctcttgtcaagaattttacaaagtttagctggcggttcttcatcagtttggtcttggagactctcagaggaattgttttctgtctctatatcataatcctcagaaatcgcatgcacttctacagcaattggaacatcttcagcagtgtgaacttctataggactctcctcttgggtttgctggttgactgattcaggtgagtcacactcttcatcacaaattacaatatcagcagatttttctgtagaaaaggcagtgtggtctagaattctaagtacaggactgggaaccaggtagttctgatttctgtttctggccttgattccatctgcaaattttggcaagtcatttgacgtctcggtatcagaatcatcatctttgttgtcaaaatattttaaatctggctgtctcatagaacagacactgtaacaatgatcagagaaaattccattgaatccatctgcaattctgcttattccagaggaatctgaataacgagaagggtgtagagtcttcctttttctttttttaggatactcattcatatcttttcaatttggtataattcttactactggagtgaggaaaaatgaattacaataagtttctgtagacagtaaaaaatgccttctatagttctttttttttgagacagtctcatgcctgacctatagttaaatctcgccgggtgcagtggttcacgcctgtaatcccagcactttgggaggccgaggcgaacagatcacctgaggtcgggaattcaagactagcctgaccaacatggggaaaccccgtctcgactgaaaatacaaaattagccgggcgtggtggcacatgcctgtaatctgagctactcgggaggctgaggcatgagaatcgcttgaatccgggaggcggaggttgtggtgacccgagatcacatcattgtcctccagcctgggtaacaggagtgaaactctgtcagtcagtcccccgaggccctcccggccggcccacgcagaggcggcggcggccgagagcgcaggcggaggggccgcgcggtccttcccgcggacgcacggcggcgggcagcgctgctccggccctagcgctcccggacgctgtgctgggccgacccctctccctccccgcgcgccccacgccctgagcgccaggcccctggcctaggctccgcggccgcactgccctggccgccacgctccgcgcctgcgccgcgcacctc

SEQ ID NO: 11221 - RNA, 1083 nt, Homo sapiens
  source 1..1083: mol_type = other RNA
ctgaatagctgggactacaggtgcccaccaccacgcccggccaattttttgtatatttagtaaagacggggtttcaccatgttagccaggatggtctcgatctcctgacctcgtgatccacccacctcggcctcccaaagtgctgggattacatgcataagccactgcgcccagcctgtaccacaaattaatggttaaaatgcatccctcatacgacaatgtaacttcttcctctcactgttgatggcctatcttcctgaaaacattaatctgcgggtgagaacttgggagatacacacagttgggttcaccataaatgaggagcctcactgacagtggaagatgcacaggaaaagaaagaagactatgggctgcttccttagaattgtcttcctgcttgctgtgttactgctagagcttcctgtgtgggctccatatggtccctattcttcccaccactcatgaaaacaccaaagagcaggttcagagtgaccacagccaagccccagctctgccagcaggcccccatcttctcctgctctgatgtggggattgtgcggttggcttgtttcctggcttctctcttcttcctggcatctctcttcatgttgctaggctcttggtgaatttgtcctgcctctgttcctccacagctccggctcctgtatgaatgcaatcccgtggcctacatcattgagcaggcaggaggcttggcgaccacggggacccagcctgtactggacgtgaagcccgaggcaattcaccagcgagtccccctcattctggggtcaccagaggatgtgcaggaatatctcacccctccagccgcgctgcaatgtccaccgccaccaccaaccgcagcgaggcgagccgcgccacggtgccgcggctcaagcctccagcatacgacctgtgactccttttcctggtcttctaagccgggcactgagcagctcaatagaaacacacggaaacctaaaaaaacaaaaacaaaaaaaacaacaacaaaaaaaacgtaactctgcttcagcattatttatatcctgaggttatgcgcatgccggttcctagactgcatgttct

SEQ ID NO: 11222 - RNA, 1118 nt, Homo sapiens
  source 1..1118: mol_type = other RNA
ctgaatagctgggactacaggtgcccaccaccacgcccggccaattttttgtatatttagtaaagacggggtttcaccatgttagccaggatggtctcgatctcctgacctcgtgatccacccacctcggcctcccaaagtgctgggattacatgcataagccactgcgcccagcctgtaccacaaattaatggttaaaatgcatccctcatacgacaatgtaacttcttcctctcactgttgatggcctatcttcctgaaaacattaatctgcgggtgagaacttgggagatacacacagttgggttcaccataaatgaggagcctcactgacagtggaagatgcacaggaaaagaaagaagactatgggctgcttccttagaattgtcttcctgcttgctgtgttactgctagagcttcctgtgtgggctccatatggtccctattcttcccaccactcatgaaaacaccaaagagcaggttcagagtgaccacagccaagccccagctctgccagcaggcccccatcttctcctgctctgatgtggggattgtgcggttggcttgtttcctggcttctctcttcttcctggcatctctcttcatgttgctaggctcttggtgaatttgtcctgcctctgttcctccacagctccggctcctgtatgaatgcaatcccgtggcctacatcattgagcaggcaggaggcttggcgaccacggggacccagcctgtactggacgtgaagcccgaggcaattcaccagcgagtccccctcattctggggtcaccagaggatgtgcaggaatatctcacctctatctatcccaaaactatcttcttcttcctacccctccagccgcgctgcaatgtccaccgccaccaccaaccgcagcgaggcgagccgcgccacggtgccgcggctcaagcctccagcatacgacctgtgactccttttcctggtcttctaagccgggcactgagcagctcaatagaaacacacggaaacctaaaaaaacaaaaacaaaaaaaacaacaacaaaaaaaacgtaactctgcttcagcattatttatatcctgaggttatgcgcatgccggttcctagactgcatgttct

SEQ ID NO: 11223 - RNA, 1203 nt, Homo sapiens
  source 1..1203: mol_type = other RNA
ctgaatagctgggactacaggtgcccaccaccacgcccggccaattttttgtatatttagtaaagacggggtttcaccatgttagccaggatggtctcgatctcctgacctcgtgatccacccacctcggcctcccaaagtgctgggattacatgcataagccactgcgcccagcctgtaccacaaattaatggttaaaatgcatccctcatacgacaatgtaacttcttcctctcactgttgatggcctatcttcctgaaaacattaatctgcgggtgagaacttgggagatacacacagttgggttcaccataaatgaggagcctcactgacagtggaagatgcacaggaaaagaaagaagactatgggctgcttccttagaattgtcttcctgcttgctgtgttactgctagagcttcctgtgtgggctccatatggtccctattcttcccaccactcatgaaaacaccaaagagcaggttcagagtgaccacagccaagccccagctctgccagcaggcccccatcttctcctgctctgatgtggggattgtgcggttggcttgtttcctggcttctctcttcttcctggcatctctcttcatgttgctaggctcttggtgaatttgtcctgcctctgttcctccacagctccggctcctgtatgaatgcaatcccgtggcctacatcattgagcaggcaggaggcttggcgaccacggggacccagcctgtactggacgtgaagcccgaggcaattcaccagcgagtccccctcattctggggtcaccagaggatgtgcaggaatatctcacctgtgtgcagaaaaatcaggcaggcagctagcgagtttgaccccacatgccctcttctgtttgtcttgcaccttgtctaaggaccctctatctatcccaaaactatcttcttcttcctacccctccagccgcgctgcaatgtccaccgccaccaccaaccgcagcgaggcgagccgcgccacggtgccgcggctcaagcctccagcatacgacctgtgactccttttcctggtcttctaagccgggcactgagcagctcaatagaaacacacggaaacctaaaaaaacaaaaacaaaaaaaacaacaacaaaaaaaacgtaactctgcttcagcattatttatatcctgaggttatgcgcatgccggttcctagactgcatgttct

SEQ ID NO: 11224 - RNA, 880 nt, Homo sapiens
  source 1..880: mol_type = other RNA
ctgaatagctgggactacaggtgcccaccaccacgcccggccaattttttgtatatttagtaaagacggggtttcaccatgttagccaggatggtctcgatctcctgacctcgtgatccacccacctcggcctcccaaagtgctgggattacatgcataagccactgcgcccagcctgtaccacaaattaatggttaaaatgcatccctcatacgacaatgtaacttcttcctctcactgttgatggcctatcttcctgaaaacattaatctgcgggtgagaacttgggagatacacacagttgggttcaccataaatgaggagcctcactgacagtggaagatgcacaggaaaagaaagaagactatgggctgcttccttagaattgtcttcctgcttgctgtgttactgctagagcttcctgtgtgggctccatatggtccctattcttcccaccactcatgaaaacaccaaagagcaggttcagagtgaccacagccaagccccagctctgccagcaggcccccatcttctcctgctctgatgtggggattgtgcggttggcttgtttcctggcttctctcttcttcctggcatctctcttcatgttgctaggctcttggtgaatttgtcctgcctctgttcctccacagctccggctcctgtatgaatgcaatcccgtggcctacatcattgagcaggcaggaggcttggcgaccacggggacccagcctgtactggacgtgaagcccgaggcaattcaccagcgagtccccctcattctggggtcaccagaggatgtgcaggaatatctcactctgcttcagcattatttatatcctgaggttatgcgcatgccggttcctagactgcatgttct

SEQ ID NO: 11225 - RNA, 1413 nt, Homo sapiens
  source 1..1413: mol_type = other RNA
ctgaatagctgggactacaggtgcccaccaccacgcccggctaattttgtgtatttttagtagagatggggtttcacggtgttagccaggacggtctcgatctcctgacctcgtgatccgcccgccttggcctcccaaagtgctgccagaagtattctttactggcttgacctttgtccccagatacgtaaatatatttatgtaacgaatctccctgacagtagaaaatgtgtaatttccaatctgaataaaactgagctatatctgaataactgagaagagtatgatattactttgattattttaaaagtgaaagggaaaatatctaaaaattggatatcgatgatacttctagacacttgattatgtagttcttgattaatttctcgttcgcaggatccagaagataaaagtgaccccctggaagctggtaaattttagcatttccactggttacatctttccaggcttccatgtcctttgctatgtcttcagatccaacaaaacatgtcaagtcacaggaaagaacagccttagatggtacgttagaggtgcaacttctaacaatgttcagatctgcccttatgatgggactacattgtttcacaaattccttggcttcagcaaaatgcttgggggtgcctccaaattccataaggtaatgacttatttgttcttctgacaattcatcatctttgggaatgcgatgccaggcctttgaatgtacaggagttgcacttgacaaaaataaatgcaatggttctggttgattgttttcttttagacctagtgcagtcctaaaagcaatgtaggatcccatactgtggccaaaaaatgcaaatggtttatcctggatgactggctgcagagcacaaacaacttcatcaactaactgggagatgtcattttcaagaggttcttcaactctgctttctcttccaggaagccttaaggagtgcacttccagcaaatcatgagtatcttggccccatttggcaaaatgagtggagccacctcccatccagggaaagcaaatcagcttaaaagttgcctcagggtttttgtataagcagttgaaaatgttttcattcctggttctcttaggttggtctcctctctccatgctgtgaggtgaggttgcaagatggctggtctctgtggcgtgttgagtgctcaacagaagtcagttcctcttgagacgaagaacctctgctcggccttatgcacacagaagagtgagtagatttctttttaaaggcgctgactcttattgacctctccaatccatatgacaacgtgaggtctcacaataggccatctgcaggctgaggagcaaggaagccagtcagagtcccagaactgaagaaattggagtctgatgttcaagggcgggaagcatccagcatgggagaa

SEQ ID NO: 11226 - RNA, 1330 nt, Homo sapiens
  source 1..1330: mol_type = other RNA
ctgaatagctgggactacaggtgcccaccaccacgcccggctaattttgtgtatttttagtagagatggggtttcacggtgttagccaggacggtctcgatctcctgacctcgtgatccgcccgccttggcctcccaaagtgctgccagaagtattctttactggcttgacctttgtccccagatacgtaaatatatttatgtaacgaatctccctgacagtagaaaatgtgtaatttccaatctgaataaaactgagctatatctgaataactgagaagagtatgatattactttgattattttaaaagtgaaagggaaaatatctaaaaattggatatcgatgatacttctagacacttgattatgtagttcttgattaatttctcgttcgcaggatccagaagataaaagtgaccccctggaagctggtaaattttagcatttccactggttacatctttccaggcttccatgtcctttgctatgtcttcagatccaacaaaacatgtcaagtcacaggaaagaacagccttagatggtacgttagaggtgcaacttctaacaatgttcagatctgcccttatgatgggactacattgtttcacaaattccttggcttcagcaaaatgcttgggggtgcctccaaattccataaggtaatgacttatttgttcttctgacaattcatcatctttgggaatgcgatgccaggcctttgaatgtacaggagttgcacttgacaaaaataaatgcaatggttctggttgattgttttcttttagacctagtgcagtcctaaaagcaatgtaggatcccatactgtggccaaaaaatgcaaatggtttatcctggatgactggctgcagagcacaaacaacttcatcaactaactgggagatgtcattttcaagaggttcttcaactctgctttctcttccaggaagccttaaggagtgcacttccagcaaatcatgagtatcttggccccatttggcaaaatgagtggagccacctcccatccagggaaagcaaatcagcttaaaagttgcctcagggtttttgtataagcagttgaaaatgttttcattcctggttctcttaggttggtctcctctctccatgctgtgaggtgaggttgcaagatggctggtctctgtggcgtgttgagtgctcaacagaagtcagttcctcttgagacgaagaacctctgctcggccttatgcacacagaagagtgagtagatttctttttaaaggcgctgactcttattgacctctccaatccttgccaggctttgagatgaactctgagcagacaatctgaaagat

SEQ ID NO: 11227 - RNA, 1501 nt, Homo sapiens
  source 1..1501: mol_type = other RNA
ctgaatagctgggactacaggtgcccaccaccacgcccggctaattttgtgtatttttagtagagatggggtttcacggtgttagccaggacggtctcgatctcctgacctcgtgatccgcccgccttggcctcccaaagtgctgccagaagtattctttactggcttgacctttgtccccagatacgtaaatatatttatgtaacgaatctccctgacagtagaaaatgtgtaatttccaatctgaataaaactgagctatatctgaataactgagaagagtatgatattactttgattattttaaaagtgaaagggaaaatatctaaaaattggatatcgatgatacttctagacacttgattatgtagttcttgattaatttctcgttcgcaggatccagaagataaaagtgaccccctggaagctggtaaattttagcatttccactggttacatctttccaggcttccatgtcctttgctatgtcttcagatccaacaaaacatgtcaagtcacaggaaagaacagccttagatggtacgttagaggtgcaacttctaacaatgttcagatctgcccttatgatgggactacattgtttcacaaattccttggcttcagcaaaatgcttgggggtgcctccaaattccataaggtaatgacttatttgttcttctgacaattcatcatctttgggaatgcgatgccaggcctttgaatgtacaggagttgcacttgacaaaaataaatgcaatggttctggttgattgttttcttttagacctagtgcagtcctaaaagcaatgtaggatcccatactgtggccaaaaaatgcaaatggtttatcctggatgactggctgcagagcacaaacaacttcatcaactaactgggagatgtcattttcaagaggttcttcaactctgctttctcttccaggaagccttaaggagtgcataaaaaaaattagaatccagaatagaccaagaattttggccaggcacggtggctcacgcctacggtggctcacgccagcacatgggtaggctgaagcaggaggatcacttgagcgccggagtttgagaccagccttggcaacatggtgagatgctgtctcttccagcaaatcatgagtatcttggccccatttggcaaaatgagtggagccacctcccatccagggaaagcaaatcagcttaaaagttgcctcagggtttttgtataagcagttgaaaatgttttcattcctggttctcttaggttggtctcctctctccatgctgtgaggtgaggttgcaagatggctggtctctgtggcgtgttgagtgctcaacagaagtcagttcctcttgagacgaagaacctctgctcggccttatgcacacagaagagtgagtagatttctttttaaaggcgctgactcttattgacctctccaatccgtatatacagacagacaaagatgcaacatttccagactctagccatgaaacaagcc

SEQ ID NO: 11228 - RNA, 1489 nt, Homo sapiens
  source 1..1489: mol_type = other RNA
ctgaatagctgggactacaggtgcccaccaccacgcccggctaattttgtgtatttttagtagagatggggtttcacggtgttagccaggacggtctcgatctcctgacctcgtgatccgcccgccttggcctcccaaagtgctgccagaagtattctttactggcttgacctttgtccccagatacgtaaatatatttatgtaacgaatctccctgacagtagaaaatgtgtaatttccaatctgaataaaactgagctatatctgaataactgagaagagtatgatattactttgattattttaaaagtgaaagggaaaatatctaaaaattggatatcgatgatacttctagacacttgattatgtagttcttgattaatttctcgttcgcaggatccagaagataaaagtgaccccctggaagctggtaaattttagcatttccactggttacatctttccaggcttccatgtcctttgctatgtcttcagatccaacaaaacatgtcaagtcacaggaaagaacagccttagatggtacgttagaggtgcaacttctaacaatgttcagatctgcccttatgatgggactacattgtttcacaaattccttggcttcagcaaaatgcttgggggtgcctccaaattccataaggtaatgacttatttgttcttctgacaattcatcatctttgggaatgcgatgccaggcctttgaatgtacaggagttgcacttgacaaaaataaatgcaatggttctggttgattgttttcttttagacctagtgcagtcctaaaagcaatgtaggatcccatactgtggccaaaaaatgcaaatggtttatcctggatgactggctgcagagcacaaacaacttcatcaactaactgggagatgtcattttcaagaggttcttcaactctgctttctcttccaggaagccttaaggagtgcataaaaaaaattagaatccagaatagaccaagaattttggccaggcacggtggctcacgcctacggtggctcacgccagcacatgggtaggctgaagcaggaggatcacttgagcgccggagtttgagaccagccttggcaacatggtgagatgctgtctcttccagcaaatcatgagtatcttggccccatttggcaaaatgagtggagccacctcccatccagggaaagcaaatcagcttaaaagttgcctcagggtttttgtataagcagttgaaaatgttttcattcctggttctcttaggttggtctcctctctccatgctgtgaggtgaggttgcaagatggctggtctctgtggcgtgttgagtgctcaacagaagtcagttcctcttgagacgaagaacctctgctcggccttatgcacacagaagagtgagtagatttctttttaaaggcgctgactcttattgacctctccaatccttgccaggctttgagatgaactctgagcagacaatctgaaagat

SEQ ID NO: 11229 - RNA, 1511 nt, Homo sapiens
  source 1..1511: mol_type = other RNA
ctgaatagctgggactacaggtgcccaccaccacgcctggctaatttttcgtatttttagtagagacggggtttcaccatgttagccaggatggtctccatctcctgacctcgtgatccacccgccttggcctcccaaagtgctgggatcacaggcgtgagccattgcactgggcctccaatgctttcgatggaaaataaaataaaataaaggcctaacagtgtggtaatgtttacttctctgccacaacactcagtatgcccctttggatctggcaacaatttaacataaggaaagactttagaccttcacaccctttcagtgagaaaaaaaaaaatgaccttagctcaaactttccacaaagctgaacagtctcattaaaacatcactccaaccttatcttaggtgggtctgtgcaaaggcctcaaggccatgtgtcttgcaggtctccatgccctgcactgcccagctctggtctctacactgcagaggagatctctattttcatgtttgaagaccatgaaccctctgcttctgaatcaaagggggaaaaactgcaaaagaagccatgtgctcaaagaaaagaatgccaaagggtataagtggcttgtgaagaagtttcacaaagctgtctccatttgctaaagctataaacagttcttgatctagtcaattgcaaaatacatggatggccagggcttctgtttaagcaaaagaagaaaaaatatcaatagcacaaaactgcccttatagtttttgaaaaaatatatctattaagataacaattttgatttttttaataagctgtgcattaagtacactttgtttccatcactctccattactctagagctccgctttgtctgcctgggccgggctggcgaccccactgcctccctcggcggtgccactgctatccgcaggtgtaaaagacaaggcagccgaatttatgcagtatcttttcccagttggacgaggcccatcatcaaaaatgtgcccaaggtgagcaccacactgagagcagcttgtttccaccctgtgcatcccataggaaaagtcatctgtgaatgtgattgcctcagaattgatcacatcgtggaatgaaggccaacctgaaccggagtcaaatttggtttctgacttaaacaatggagttccacaaacaacacatttatatattccaggatctttgtgatgtgtgtattctccttcaaaggcactttcggtccctttctcctgagtgacatggtactgcaggggtgttagccgcttcctcagttcctgctgggaaaagaccaccttacagttctttttatccctacacgacccggactgcgcacttcccagagccgcggccaggcagaggcagaggcagagggagaggcagagcgagagggggcgcgggagggtccgccgcgggctcatggaaaggccaggcagccgccgccggtgtccgaacctcgctccctccctccccggctccgggcgacggacggggcggcgggaggcat

SEQ ID NO: 11230 - RNA, 1638 nt, Homo sapiens
  source 1..1638: mol_type = other RNA
ctgaatagctgggactacaggtgcccaccaccacgcctggctaatttttcgtatttttagtagagacggggtttcaccatgttagccaggatggtctccatctcctgacctcgtgatccacccgccttggcctcccaaagtgctgggatcacaggcgtgagccattgcactgggcctccaatgctttcgatggaaaataaaataaaataaaggcctaacagtgtggtaatgtttacttctctgccacaacactcagtatgcccctttggatctggcaacaatttaacataaggaaagactttagaccttcacaccctttcagtgagaaaaaaaaaaatgaccttagctcaaactttccacaaagctgaacagtctcattaaaacatcactccaaccttatcttaggtgggtctgtgcaaaggcctcaaggccatgtgtcttgcaggtctccatgccctgcactgcccagctctggtctctacactgcagaggagatctctattttcatgtttgaagaccatgaaccctctgcttctgaatcaaagggggaaaaactgcaaaagaagccatgtgctcaaagaaaagaatgccaaagggtataagtggcttgtgaagaagtttcacaaagctgtctccatttgctaaagctataaacagttcttgatctagtcaattgcaaaatacatggatggccagggcttctgtttaagcaaaagaagaaaaaatatcaatagcacaaaactgcccttatagtttttgaaaaaatatatctattaagataacaattttgatttttttaataagctgtgcattaagtacactttgtttccatcactctccattactctagagctccgctttgtctgcctgggccgggctggcgaccccactgcctccctcggcggtgccactgctatccgcaggtgtaaaagacaaggcagccgaatttatgcagtatcttttcccagttggacgaggcccatcatcaaaaatgtgcccaaggtgagcaccacactgagagcagcttgtttccaccctgtgcatcccataggaaaagtcatctgtgaatgtgattgcctcagaattgatcacatcgtggaatgaaggccaacctgaaccggagtcaaatttggtttctgacttaaacaatggagttccacaaacaacacatttatatattccaggatctttgtgatgtgtgtattctccttcaaaggcactttcggtccctttctcctgagtgacatggtactgcaggggtgttagccgcttcctcagttcctgctgggaaaagaccaccttacagttctttttatccctacacgaccctgagggaagcccacaggctcgaagggctactggctggctctttgtcaccaaatgcagcaggttgaatgcagacatcactgtgatatcttcaccaacaaaacgagaagcaaagaacaggggcaagagcggactgcgcacttcccagagccgcggccaggcagaggcagaggcagagggagaggcagagcgagagggggcgcgggagggtccgccgcgggctcatggaaaggccaggcagccgccgccggtgtccgaacctcgctccctccctccccggctccgggcgacggacggggcggcgggaggcat

SEQ ID NO: 11231 - RNA, 1570 nt, Homo sapiens
  source 1..1570: mol_type = other RNA
ctgaatagctgggactacaggtgcccaccaccacgcctggctaatttttcgtatttttagtagagacggggtttcaccatgttagccaggatggtctccatctcctgacctcgtgatccacccgccttggcctcccaaagtgctgggatcacaggcgtgagccattgcactgggcctccaatgctttcgatggaaaataaaataaaataaaggcctaacagtgtggtaatgtttacttctctgccacaacactcagtatgcccctttggatctggcaacaatttaacataaggaaagactttagaccttcacaccctttcagtgagaaaaaaaaaaatgaccttagctcaaactttccacaaagctgaacagtctcattaaaacatcactccaaccttatcttaggtgggtctgtgcaaaggcctcaaggccatgtgtcttgcaggtctccatgccctgcactgcccagctctggtctctacactgcagaggagatctctattttcatgtttgaagaccatgaaccctctgcttctgaatcaaagggggaaaaactgcaaaagaagccatgtgctcaaagaaaagaatgccaaagggtataagtggcttgtgaagaagtttcacaaagctgtctccatttgctaaagctataaacagttcttgatctagtcaattgcaaaatacatggatggccagggcttctgtttaagcaaaagaagaaaaaatatcaatagcacaaaactgcccttatagtttttgaaaaaatatatctattaagataacaattttgatttttttaataagctgtgcattaagtacactttgtttccatcactctccattactctagagctccgctttgtctgcctgggccgggctggcgaccccactgcctccctcggcggtgccactgctatccgcaggtgtaaaagacaaggcagccgaatttatgcagtatcttttcccagttggacgaggcccatcatcaaaaatgtgcccaaggtgagcaccacactgagagcagcttgtttccaccctgtgcatcccataggaaaagtcatctgtgaatgtgattgcctcagaattgatcacatcgtggaatgaaggccaacctgaaccggagtcaaatttggtttctgacttaaacaatggagttccacaaacaacacatttatatattccaggatctttgtgatgtgtgtattctccttcaaaggcactttcggtccctttctcctgagtgacatggtactgcaggggtgttagccgcttcctcagttcctgctgggaaaagaccaccttacagttctttttatccctacacgaccctgagggaagcccacaggctcgaagggctactggctggctctttgtcaccaaatgcagcaggttgaatgcagacatcactgtgatatcttcaccaacaaaacgagaagcaaagaacaggggcaagagctccttccgttcggcccctcaccgctggcgcggggcgcaacccttctgctccccttctcggctgaggcaggggctgtccccgcaggtggccgagggggcgcagcaggcgcagaat

SEQ ID NO: 11232 - RNA, 1876 nt, Homo sapiens
  source 1..1876: mol_type = other RNA
ctgaatagctgggactacaggtgcccaccaccacgcctggctaatttttcgtatttttagtagagacggggtttcaccatgttagccaggatggtctccatctcctgacctcgtgatccacccgccttggcctcccaaagtgctgggatcacaggcgtgagccattgcactgggcctccaatgctttcgatggaaaataaaataaaataaaggcctaacagtgtggtaatgtttacttctctgccacaacactcagtatgcccctttggatctggcaacaatttaacataaggaaagactttagaccttcacaccctttcagtgagaaaaaaaaaaatgaccttagctcaaactttccacaaagctgaacagtctcattaaaacatcactccaaccttatcttaggtgggtctgtgcaaaggcctcaaggccatgtgtcttgcaggtctccatgccctgcactgcccagctctggtctctacactgcagaggagatctctattttcatgtttgaagaccatgaaccctctgcttctgaatcaaagggggaaaaactgcaaaagaagccatgtgctcaaagaaaagaatgccaaagggtataagtggcttgtgaagaagtttcacaaagctgtctccatttgctaaagctataaacagttcttgatctagtcaattgcaaaatacatggatggccagggcttctgtttaagcaaaagaagaaaaaatatcaatagcacaaaactgcccttatagtttttgaaaaaatatatctattaagataacaattttgatttttttaataagctgtgcattaagtacactttgtttccatcactctccattactctagagctccgctttgtctgcctgggccgggctggcgaccccactgcctccctcggcggtgccactgctatccgcaggtgtaaaagacaaggcagccgaatttatgcagtatcttttcccagttggacgaggcccatcatcaaaaatgtgcccaaggtgagcaccacactgagagcagcttgtttccaccctgtgcatcccataggaaaagtcatctgtgaatgtgattgcctcagaattgatcacatcgtggaatgaaggccaacctgaaccggagtcaaatttggtttctgacttaaacaatggagttccacaaacaacacatttatatattccaggatctttgtgatgtgtgtattctccttcaaaggcactttcggtccctttctcctgagtgacatggtactgcaggggtgttagccgcttcctcagttcctgctgggaaaagaccaccttacagttctttttatccctacacgaccctgagggaagcccacaggctcgaagggctactggctggctctttgtcaccaaatgcagcaggttgaatgcagacatcactgtgatatcttcaccaacaaaacgagaagcaaagaacaggggcaagagctggcaaactcggggttctgttcgattttggcctgtgaaatgccaggcgggcccgctggagtctggcccagcagcggggcagcagcgcagggagggcgggcggcgggtgcgctcccgggtgcgcccctccctgccgcctgcccgccgccccgcacccccgtcctctccgaggcgcgcggcgaaaagcgcaggcctggcgggccggttcccacgcctcgggcccgttatctgagcggcaaccccggcagggtcgacgcacagagcagagggctccgggatggacccctcccctgcctcccgcgggctgccccgccagatccctctctcctgggcccgcgcggggcgagaggctcccgcgggttcaggttcgctcccgggacaggataaggtgtcagtgaggctgccagacgcctcccttcgg

SEQ ID NO: 11233 - RNA, 1744 nt, Homo sapiens
  source 1..1744: mol_type = other RNA
ctgaatagctgggactacaggtgcccaccaccacgcctggctaatttttcgtatttttagtagagacggggtttcaccatgttagccaggatggtctccatctcctgacctcgtgatccacccgccttggcctcccaaagtgctgggatcacaggcgtgagccattgcactgggcctccaatgctttcgatggaaaataaaataaaataaaggcctaacagtgtggtaatgtttacttctctgccacaacactcagtatgcccctttggatctggcaacaatttaacataaggaaagactttagaccttcacaccctttcagtgagaaaaaaaaaaatgaccttagctcaaactttccacaaagctgaacagtctcattaaaacatcactccaaccttatcttaggtgggtctgtgcaaaggcctcaaggccatgtgtcttgcaggtctccatgccctgcactgcccagctctggtctctacactgcagaggagatctctattttcatgtttgaagaccatgaaccctctgcttctgaatcaaagggggaaaaactgcaaaagaagccatgtgctcaaagaaaagaatgccaaagggtataagtggcttgtgaagaagtttcacaaagctgtctccatttgctaaagctataaacagttcttgatctagtcaattgcaaaatacatggatggccagggcttctgtttaagcaaaagaagaaaaaatatcaatagcacaaaactgcccttatagtttttgaaaaaatatatctattaagataacaattttgatttttttaataagctgtgcattaagtacactttgtttccatcactctccattactctagagctccgctttgtctgcctgggccgggctggcgaccccactgcctccctcggcggtgccactgctatccgcaggtgtaaaagacaaggcagccgaatttatgcagtatcttttcccagttggacgaggcccatcatcaaaaatgtgcccaaggtgagcaccacactgagagcagcttgtttccaccctgtgcatcccataggaaaagtcatctgtgaatgtgattgcctcagaattgatcacatcgtggaatgaaggccaacctgaaccggagtcaaatttggtttctgacttaaacaatggagttccacaaacaacacatttatatattccaggatctttgtgatgtgtgtattctccttcaaaggcactttcggtccctttctcctgagtgacatggtactgcaggggtgttagccgcttcctcagttcctgctgggaaaagaccaccttacagttctttttatccctacacgaccctgagggaagcccacaggctcgaagggctactggctggctctttgtcaccaaatgcagcaggttgaatgcagacatcactgtgatatcttcaccaacaaaacgagaagcaaagaacaggggcaagagttagcaaagctgcagtctcactgtgcttccacagctgaccataaaacgtcttcctattctgtttcatcaactcctgtaccaggcagcctgggcgcctaccaaccacggtggccatctggcttatgtcaaagccagcgcacaggaagagaggcagtgatgtcactcaggcatggtggtgggcgcctgcaatcccagctactcaggaggctgaggcaggagaatcgcttgaacctgggaggcagagattacagtgacctgagattgcgtactgcactccagcctgggcaac

SEQ ID NO: 11234 - RNA, 1802 nt, Homo sapiens
  source 1..1802: mol_type = other RNA
ctgaatagctgggactacaggtgcccaccaccacgcctggctaatttttcgtatttttagtagagacggggtttcaccatgttagccaggatggtctccatctcctgacctcgtgatccacccgccttggcctcccaaagtgctgggatcacaggcgtgagccattgcactgggcctccaatgctttcgatggaaaataaaataaaataaaggcctaacagtgtggtaatgtttacttctctgccacaacactcagtatgcccctttggatctggcaacaatttaacataaggaaagactttagaccttcacaccctttcagtgagaaaaaaaaaaatgaccttagctcaaactttccacaaagctgaacagtctcattaaaacatcactccaaccttatcttaggtgggtctgtgcaaaggcctcaaggccatgtgtcttgcaggtctccatgccctgcactgcccagctctggtctctacactgcagaggagatctctattttcatgtttgaagaccatgaaccctctgcttctgaatcaaagggggaaaaactgcaaaagaagccatgtgctcaaagaaaagaatgccaaagggtataagtggcttgtgaagaagtttcacaaagctgtctccatttgctaaagctataaacagttcttgatctagtcaattgcaaaatacatggatggccagggcttctgtttaagcaaaagaagaaaaaatatcaatagcacaaaactgcccttatagtttttgaaaaaatatatctattaagataacaattttgatttttttaataagctgtgcattaagtacactttgtttccatcactctccattactctagagctccgctttgtctgcctgggccgggctggcgaccccactgcctccctcggcggtgccactgctatccgcaggtgtaaaagacaaggcagccgaatttatgcagtatcttttcccagttggacgaggcccatcatcaaaaatgtgcccaaggtgagcaccacactgagagcagcttgtttccaccctgtgcatcccataggaaaagtcatctgtgaatgtgattgcctcagaattgatcacatcgtggaatgaaggccaacctgaaccggagtcaaatttggtttctgacttaaacaatggagttccacaaacaacacatttatatattccaggatctttgtgatgtgtgtattctccttcaaaggcactttcggtccctttctcctgagtgacatggtactgcaggggtgttagccgcttcctcagttcctgctgggaaaagaccaccttacagttctttttatccctacacgaccctgagggaagcccacaggctcgaagggctactggctggctctttgtcaccaaatgcagcaggttgaatgcagacatcactgtgatatcttcaccaacaaaacgagaagcaaagaacaggggcaagagttagcaaagctgcagtctcactgtgcttccacagctgaccataaaacgtcttcctattctgtttcatcaactcctgtaccaggcagcctgggcgcctaccaaccacggtggccatctggcttatgtcaaagccagcgcacaggaagagaggcagtgatgtcactcggactgcgcacttcccagagccgcggccaggcagaggcagaggcagagggagaggcagagcgagagggggcgcgggagggtccgccgcgggctcatggaaaggccaggcagccgccgccggtgtccgaacctcgctccctccctccccggctccgggcgacggacggggcggcgggaggcat

SEQ ID NO: 11235 - RNA, 1760 nt, Homo sapiens
  source 1..1760: mol_type = other RNA
ctgaatagctgggactacaggtgcccaccaccacgcctggctaatttttcgtatttttagtagagacggggtttcaccatgttagccaggatggtctccatctcctgacctcgtgatccacccgccttggcctcccaaagtgctgggatcacaggcgtgagccattgcactgggcctccaatgctttcgatggaaaataaaataaaataaaggcctaacagtgtggtaatgtttacttctctgccacaacactcagtatgcccctttggatctggcaacaatttaacataaggaaagactttagaccttcacaccctttcagtgagaaaaaaaaaaatgaccttagctcaaactttccacaaagctgaacagtctcattaaaacatcactccaaccttatcttaggtgggtctgtgcaaaggcctcaaggccatgtgtcttgcaggtctccatgccctgcactgcccagctctggtctctacactgcagaggagatctctattttcatgtttgaagaccatgaaccctctgcttctgaatcaaagggggaaaaactgcaaaagaagccatgtgctcaaagaaaagaatgccaaagggtataagtggcttgtgaagaagtttcacaaagctgtctccatttgctaaagctataaacagttcttgatctagtcaattgcaaaatacatggatggccagggcttctgtttaagcaaaagaagaaaaaatatcaatagcacaaaactgcccttatagtttttgaaaaaatatatctattaagataacaattttgatttttttaataagctgtgcattaagtacactttgtttccatcactctccattactctagagctccgctttgtctgcctgggccgggctggcgaccccactgcctccctcggcggtgccactgctatccgcaggtgtaaaagacaaggcagccgaatttatgcagtatcttttcccagttggacgaggcccatcatcaaaaatgtgcccaaggtgagcaccacactgagagcagcttgtttccaccctgtgcatcccataggaaaagtcatctgtgaatgtgattgcctcagaattgatcacatcgtggaatgaaggccaacctgaaccggagtcaaatttggtttctgacttaaacaatggagttccacaaacaacacatttatatattccaggatctttgtgatgtgtgtattctccttcaaaggcactttcggtccctttctcctgagtgacatggtactgcaggggtgttagccgcttcctcagttcctgctgggaaaagaccaccttacagttctttttatccctacacgaccctgagggaagcccacaggctcgaagggctactggctggctctttgtcaccaaatgcagcaggttgaatgcagacatcactgtgatatcttcaccaacaaaacgagaagcaaagaacaggggcaagagttagcaaagctgcagtctcactgtgcttccacagctgaccataaaacgtcttcctattctgtttcatcaactcctgtaccaggcagcctgggcgcctaccaaccacggtggccatctggcttatgtcaaagccagcgcacaggaagagaggcagtgatgtcactctccttccgttcggcccctcaccgctggcgcggggcgcaacccttctgctccccttctcggctgaggcaggggctgtccccgcaggtggccgagggggcgcagcaggcgcagaatggaatcccggctcggggtcacaccct

SEQ ID NO: 11236 - RNA, 1647 nt, Homo sapiens
  source 1..1647: mol_type = other RNA
ctgaatagctgggactacaggtgcccaccaccacgcctggctaatttttcgtatttttagtagagacggggtttcaccatgttagccaggatggtctccatctcctgacctcgtgatccacccgccttggcctcccaaagtgctgggatcacaggcgtgagccattgcactgggcctccaatgctttcgatggaaaataaaataaaataaaggcctaacagtgtggtaatgtttacttctctgccacaacactcagtatgcccctttggatctggcaacaatttaacataaggaaagactttagaccttcacaccctttcagtgagaaaaaaaaaaatgaccttagctcaaactttccacaaagctgaacagtctcattaaaacatcactccaaccttatcttaggtgggtctgtgcaaaggcctcaaggccatgtgtcttgcaggtctccatgccctgcactgcccagctctggtctctacactgcagaggagatctctattttcatgtttgaagaccatgaaccctctgcttctgaatcaaagggggaaaaactgcaaaagaagccatgtgctcaaagaaaagaatgccaaagggtataagtggcttgtgaagaagtttcacaaagctgtctccatttgctaaagctataaacagttcttgatctagtcaattgcaaaatacatggatggccagggcttctgtttaagcaaaagaagaaaaaatatcaatagcacaaaactgcccttatagtttttgaaaaaatatatctattaagataacaattttgatttttttaataagctgtgcattaagtacactttgtttccatcactctccattactctagagctccgctttgtctgcctgggccgggctggcgaccccactgcctccctcggcggtgccactgctatccgcaggtgtaaaagacaaggcagccgaatttatgcagtatcttttcccagttggacgaggcccatcatcaaaaatgtgcccaaggtgagcaccacactgagagcagcttgtttccaccctgtgcatcccataggaaaagtcatctgtgaatgtgattgcctcagaattgatcacatcgtggaatgaaggccaacctgaaccggagtcaaatttggtttctgacttaaacaatggagttccacaaacaacacatttatatattccaggatctttgtgatgtgtgtattctccttcaaaggcactttcggtccctttctcctgagtgacatggtactgcaggggtgttagccgcttcctcagttcctgctgggaaaagaccaccttacagttctttttatccctacacgaccctgagggaagcccacaggctcgaagggctactggctggctctttgtcaccaaatgcagcaggttgaatgcagacatcactgtgatatcttcaccaacaaaacgagaagcaaagaacaggggcaagagttagcaaagctgcagtctcactgtgcttccacagctgaccataaaacgtcttcctattctgtttcatcaactcctgtaccaggcagcctgggcgcctaccaaccacggtggccatctggcttatgtcaaagccagcgcacaggaagagaggcagtgatgtcactctggcaaactcggggttctgttcgattt

SEQ ID NO: 11237 - RNA, 1316 nt, Homo sapiens
  source 1..1316: mol_type = other RNA
ctgaatagctgggactacaggtgcccaccaccacgcctggctaattttttatatttttagtagagacagggtttcaccatgttagccaagatggtctcgatctcctgacctcgtgatccgcccacctgggcctcccaaagtgctgggattacaggcgtgagcccccgcacccggccaaaggcaggattatttgttaagcgggttgcagtgttctaccagaccccccaccctcaacccaagcccctggtctcactgggacttggccactgccaggagcgtctggcccttcacggcttcaggcccagcacagcgcgtgtcattctgggaaaacatcttgtctttttgggcctgaagccaacgatagaggtcgctcaggttctggtcacagatccaggggttgccggagatgtcgaagccatcccgcatgtcccagtttggctgccctagggatgcccagagcccctcgggcacgctggccagtgagttattggagaggtccagcatgtccagctgccgcaggccctggaaggcaccggctgccaccctggccagcttgttgccgttcaggaagaggtagcgcaggtccggctgcggcaagaggagatcttttcccagtacttgcaatttgttgccttctagatgtagccgttctaattgcagcggacccctcaggaggtcaggtggcaaggtctccaactggttctccccaaggtcaagggtgcgcaggagggtgaagttggccagcagcccggggggcagtttccggaggcggttcccagacaggtccagatgccccagagctttcaggccgtgtagccacgagacctccaggacctccagctggttttctttcaataccagggtgtccagggtggctgaggcctggaagaggcccgggggcagcccggtcagggcgtttcgggttagatccagcaccctcagctgcggcactggccgcaggaattcgggcgagaggctttccagcccattgctggagaggtgcaattcttggagcttagaggcgccctggaggaggttggctggcaggtgggtcaggttgaagaattccacggccaggtgcacggtgtcggctggcaggtagccggggatttcggcaggtggttgacaggagatggagctgccatggtctgagcggaacacctggcagtctttggggctcagggtgaccccccaggctgaggctgccaacagcagcagcaggaacagagttctagaaacatggggttgaatgccccctgggctttttggtcgctgtctgctccaagaggacatggtagctctgctcttttgcttct

SEQ ID NO: 11238 - RNA, 3447 nt, Homo sapiens
  source 1..3447: mol_type = other RNA
ctgaatagctgggactacaggtgcccaccaccacgcctggctaattttttgtatttttagtagagacagcatttcacagtgttagccaggatggtcttgatctcctgacctcgtgatccaccctccttggtctcccaaagtgctggggttacggcgtgagccatcacacctggccaaagttacttcttaaatacaaggatggctctttgccgtgatcatggtttccatgtttgctttcgttccatctggctttcggttactcccatttccctttcccagtctctgtgagcggtaacacttggtatcgtatagcatcatctgcgatactccaaaggaatgggcagacatgcactcctgcgcccttctaatgtccctaggaaagcagcacactgaccctgaaactgccagcacagagccacatcagcagcaggaaagacactgagtgagccagtatgtgcaatgacaggatggctttacacaaagactcggttgcatgccaagtcagggtgtaatggagcaagcccccagggcagaccatgcccactgcactctctctgagcagctgaagttctgtctctgcatgttcatcttagaaggtggcatggatgccagagtgcagcttcttccgcctgcccctaataagacagtgagtcagggctcaggtcccccaggaagaggaaactgcaatgaacgggcactttctctatcatttgtgtggcatgtaccacactgcagccacccgtgtcactgctcctgtgtaacaggattgatgttgctattttcctaatgatcctgtctactgagaaggcaggaagccacatgcctcctgcaacaaccagaagccaacaagccagtctcctctctcaacaaggtaagacaaatgatgtaaaaataggttaaattacttcgaaactttaattacagatacttttccacgcaacatttctgaaatgaaagctttgattctcccctttttttgcataaaggctgggaaggtggtttggccagaccgtacatctttttgtatatacatatctacacctgtgtctcttctttattaataaaaggtgtcttgatcacagtcccaaaccaactctgcattggattccagcatataaaactcagagagtaaaacaatttcaaaggaagacaggctgcaaccacaggaaaatggcaggaaaagttgtagcttgatagttgtttcttctaagtttaactcagaaatataataataattaagagaaaaaaataagaggccctagctttcatccctgctaccaaacacgctcgtccagaactctaggctgtcttaaagtgcaattactgttgtgaagttgctcaggccagggatcaggctggacggagttcaaagcagaaacttcaaacactccttgctgttcatgactcaggggctgggagggagggagaggagaaaaagaaggacagttctctggcattcaagtgcatcaaaagaataaatgtcttttcttttggtaaagcaaatctgtcaatagtaaggaatcctggtttggaaaaatagaactttctaaaacttctatctgcggatgttccaatgcagcagagggacaaggcaggcaagtgcagccagcagcagggaccaggtgtgcctcccaggggcccggccatacaggctgcttccactgtcttctgcgaggtcctctgccctcggcgaagaggaggcacactggaccaagggcatctggtaggacgtggctctcttctctggcctgtctgggctggacccgtcgctgggcctctgaccgttgaacagcagatagcgcccccgggcatcctgttccattttgaagatctcgtactccgtgtgaggtagtttgatgcccagggccacgcagccattggtgtgggtcacatcctgctggatgcccacctgccaggagccctcggccccgcactcattcccgttgaagacgttgagcagtgaggctgtggccgcatccatgggggtgaccttcatgtgattcactttgaacacgaactcggtgcctcccatgaccctggacgagaggacgccgcggctgtagcggccccgggcgtagatggagaaggtggggtgcttgcacaccgggtctgagtagtggtagtagtggccctcccaggtgttgttgttgtcatggaagatgaagtggcgggtgaggaagaggacttcggggcgcacctcacagcgctggctcacccactccccgtgcaggccgatggtcaggtctgcctttgggggcaggatgggagggtggtgctcgtctgaccgatagatgatccgacaggcgatgcaggcatggtcgtggttcttggcattctgcagagggggctggtaactggagggccggtagaacatcctctgggtggcatcagtgtgaatgtcaccaaggaagagctcctcgaccaggtggtcgaggttgtggtgaaggtactgcttctccacccggatgagctgaagttcatgcatggcaaagttcacggccttggtgcactcacagccgttctcctctcgccagaggtcataggccacgtcctgcacccagggacccccgtctgcgaggaagcccgggcatgtgcggttcacctgctggccgagcttctcggccaccgcctctgtgtggcagatcacctggacgttgtgcagctggtagtcggcttccgtgccccctcggatgatccaggaggcctggcggaggcggatcttgccccggatgatgagagtataagtgggatttgtgcaccggttgctgccataataaaattggtaggccttgaaggtgttattgtggtagaatctgtaggaccttgtgatgaactctgggcctgaccttacttcacagcctgtggagacccagtggccctcgattgtaggtggcatctgcactgtgatccttgcaccattgtggagatgtttgagcatgtgatggcactgtgactccttaaaagccctccaggcacttttctctaaggacctaggatgagacctgctgtctggatgaaggagggcagaaccctctcccagcccgtgaagcaggagggccgggaacaggtatctgagcaggaggcggcgcggccaggacatttccagtcctgctctggggcctcccgcacgccgcgctccgatttggtgcccgggcaactgggcgcgcgctctgccctccgcctccggccgggtgcggccgggccaggccggggcttcaggcggctgccgcgcgccccatgcccggcgggctaggcgcggggctgcggggcgcgcgctctctgggcgccgtcgggcggctgtgggcgccccggcccggtccgcgtcccggcctctctgccgcccgccccgacttctccgcgcccggccccgcgtcccgccccggccgccgcgtgcgccgctctgagctgcagtggccgccaccgccaccgcagctgcagcgtctcttc

SEQ ID NO: 11239 - RNA, 5335 nt, Homo sapiens
  source 1..5335: mol_type = other RNA
ctgaatagctgggactacaggtgcccaccaccacgcctggttaattttttatacttttagtagagatggggtttcaccgtgttagccaggatggtctcgatctcctgacctcgtgatccacgcacctcggcctcccaaagtgctgggattacaggcgtgagccataccttgcccagccttgtcacaaaaaaatatttaacatgatacaataagcaaagaagggaggagaacactcttggaaacagtggaaatgtttacagtgtagattgtggttatggtttgacagaggtatgcttagctccaaactcatcaagttgtatacattaaatatggacagccttcatatgtcagtcaggcctcaataaaatggtagaatactaacagtaataataagctgacatctgccatatatatcagtactgtgcacagggttaatgggagtctgctccagagagcgggatttgggattttgctgaacctgcatagccagtccggcccgtggactagagaagtttgcctgctggcctcatgcagctggctgtgtgatggttcccaccattgtcatccaaaccaagtctgtctgagctgagttgtgtgctgggtgacttgcctcccaaacctgttggagggggctgctgggtctagatctgtgggttagaaattgctgacacatcatcctatggtccacctgacacatctctgaccgcagtgtgacaaggcagcccgaatctgagggcaggtgagtgcccaggccaggacctaggtcctaacagatatcaagtgaacagtggttcctgttccttccctctgcctggtggggacactctcaggggaagactcaaggctgcccctcaaaggcaccagcatgcaccctacaattctgcttcatggagtcctgaatgctgggcaggaaatggcattgccggggtggggccatcttcagggagggcctccaccctccaggggtgggtctttgcatctgtgaccagcaaatcagtggctaggaggacacctgcgctggggaatagatagaaccacagtgggaggcaagccctggaagacgagctcagtgctggcgcaggagaagaaagcatcacaggacaaaggcggggacaacccatggcttggcccaggttaaaaaccatccagcttcacgatcagctcacggacagcaagcgaagtggccattcactggtgcaccaggaaattcggggcctgtcacttggttctctctgttctcagaagcaggggcaccttttttcacatttaagacagaagagacacagaaaaatcaaagcaaagacacagagcgcggaaaatgccaggacaaagaccagcacgtgctcagcatgaagcatgggtgggccgggcctgaggcgacagggagacctgggcatgcatttccctagaatgaagactctgcctacactaagatatctcctattacaactgtacagttcaaaaggcagaggtacacagcaaaaccagtcattgcactactgctcacagtagagacaatttggaagcaacctaaaggagcattgaagacacccagtgaacaaaatgtgggacccatacataggatgaaattacaggcaatcataaatgatgttacatccgaaggtttgataagaaaacatgtttctaaggtgttgttaaatggaaaagaaatgttttcaaagctgttcatgaactatgatcctatttggaccaaaggaaataaaaggtagaaatgtgtgtctacacacagagaaaagaatggcagttaatattacaaaatatgaacagcgtttgcatctgagcactggcataatgggttgttctatcttctcttttttgtgtgtattttccaaattgtatgctgaaaacatgtatcagttttatgttctggaacaaaataaatgtttttgtttcatccttcaaatcccatggagtggaatcctagttagagctttcaaatcttttgcattaaatcaccccctgggtgaactgaggcagcccaagcaggtacgatttatctctactttatggctggggaaggcggggagcaagctgagaccatgccctgcccagaacagatgggtgctccgtggctctccagggctcgctgtccactggtgcagccaagtgcagatgggcaggaagcagaggagggtgcagaatccacggcgagaagagcccctctggcccggcctcccgtgcggtctcatctgtgtcctccttagacagggctgaggatccacagctcaggtgcccatctggctccctgccctgttctggggttcagcttgtgtctagtcacgtggctgttgcaccagaggttgccaggtgctgcagcagagcttccagggggctcctgtggatgacggctctttccagcaggctctggacacatcctcctctgttcctactcctggctctcctatctcagtccaataaggcttacatccctggggttcatccacgggccatgctgggtctctgggcagtggctccaggcgaggatgggccagcctggttagagagcaaggcctgggaatctgatcctggccagagctgactggggtccaggaacccaccaggagaagaatgtctgggatgagaaaggtgcccggcagatgcacaagagggctctggcccagaactcgggacccaggcacttcaccaatggccttcccctctggctaagattggaagccctctggggggattgcagagaaccacctctccaccctgacccaggcctagaagagacagcaaactcccaggactttggggaaccagcagagcccaggctgttagctgggacctggacagtcttggcatgcaggactgaggactggtgcccatccgtcaccttttgccctgacagagtcctccagccccctgcctgtcctctccctcccatgctgccctcacctgctaaccacgatgggcctggctgaccacatctcattcccagaagaaaagtctccagagggagagagttcagactcctcaaccccacactgaggatgctccatgatccccagccaagttttccaaattcatccactacaccccagctatacgttcatagcagcttaagcctctccacaatcggcctatgtccatctgtctctcccaccttgacttctgaagggcagagcccaggtcttattcatcttcatatcctgccatgccaccttggtcccctccccagcacatgaccttcaatgtacccaggaggcactcattgaagacttgttctatggaaagaataaagttgtggccaactacagattctactcctaactctgcaaaattgcagtgctgtttgctacaaagaaatttgcaggctggtgaaatgttctcggaggatcttagaccatcgaatttttcaaggctcttttttaatctccttcaattcttgaaaagactctgaccctttgaccatctgctgcgcacggagtctgctctgaatccacacaaaggcttccccatcctgcccagtctcccaaggcacaaaataaaaccagcttcggaaaatgtaaacccagagcaaggtgatccgtcactaaaatttcctgggaggaagctcaccttccgtgaccataaattgttggtgagccatctcacctattgtgcggtgctctccaaacagacacctgttgccatagcaaccctcacatctgtcgctaccttagaagagaacaccttttaaaaagaaatctacttagcaacatggcacattaacttctgcaccttcttacggactctcagaaatctaggcctgagtacgctaaggtgaatggtgcctctttgaacaatctagaagacactgcttcagccaacagtggtcccttcctccacctgcccccacctgtctctgggtatgagtcaagggctggcactgcacacagggcagttacacaagccgattgttataaaaataacgctacggttcagggtgttttgctcacagaatttcacttagtcctagggacagtctgtgcagcaagcactgtccctgcgttggtgataaggggcccagccccaaagctccagcttcctccagcgcagccttctgcctgtcatgagggtgcagccacacctggctcagggcaggccctccacacgctgtggatctgcttgtgttcccaacaacccagaaagaaagatttttttttattatccctgttttacagaggagaaagcaatcttggaggagtgacgtatctccccgagatgcctccagaagtcagcggaggcacagaggctcacactcccagctcacatttcaccagtggcttccaggctgcctcccataagcctgagaagaggcttccccgtgtggcttaggaataaattccaatctcgcaagaacagccctgtggccaggctgtcaactcttctggaattctccatggaaacatttctgcatattgcaggggatgaagaccagggaagcaggtagcagacgtacacgtgcaggaatcacctgctggatttggtgaaaatgcagatttgactcatgggtctgggcggggcctgagcagctgcattctaaccagctgccgggtgatgccgatgctctgctcctcggccgcaatttgacaaaagggacacggcgcctcctcctgggagagatgggggctctgcggtcgtggttgatgcgtttagtttgttttgctttcgcgaagtaggagctcattcactcttgattcaatccatcaggaacacgaaagcagattgtgtgcagggagagatcttatttgaattaatgctgacgactccactgccacaggacttccccttgagcagtcagccacaagtcacttcctccaggggtggccatgactctctggagcacctccaaccccatgtcacaggcagcttggccgagagaactccagctgggaaactcccgtccagtccacgcagggaatctggctctgcatctgggtgggtggcctgtgtggcatctgcctctctgtgaagcttccttgtgggttgctgggaggatcgatgagatggagccgacagaggctcgcgacaagagttcaggaaacacctgtaatggctgctgttgtgaacacatggccacaggtcccagagggttgttagggtgatccggtagcacctggagcccatcagccaactcctccaggttccttccaagggattcagacatccggggcagccaactgattcaagaaccaacagttcatagctttccaggcaatttccacagcgagaagaaaaaaggaagctcaaggcctgcaccagcgcttccgggctgggtcagaaaaacaggtcgtcctcgccgcccgcgccggcgcctgcagcaggttcc

SEQ ID NO: 11240 - RNA, 1052 nt, Homo sapiens
  source 1..1052: mol_type = other RNA
ctgaatagctgggactacaggtgcccaccaccacgtccggctaatttttttgtattttttgtagagttgaggttttaccttgttagctaggatggtctcgagctcctgacctcgtgatccacctgatgagacctctttttaggatctgtccatcagggtagttggacttcttacatgggggcacagggctccaagagaccaaagtagaagctgccagtcctcttaaagtctagaccctgaactggcataccatcactttcactgttctcgattggtcaaggcagaggccagctcagattcaaggtcaaaggaaataaaccccaccattaatgggaaggaagtgtcaggtaatttgcaaccatctttaatctgccacattactcttccatgtgctttccattgttttgttatatttttctgttgcttgtactcctcgtttttagatgatttccaagatgaagaaggaataggaagccctattatttgccatctctaaagcctggtagtttttaaggtgtctgaagataatgggtgtggtagagacagaggcaagggcagttaattagccaagacttgatgttttcctcatcttctatacagtaacttttttttttttttttttagacatagtttcactccatcatccaggctgtagtacagtggcacagtcttgactcactgcaacctctatctcccagattcaagcagtcctcctacctcagcctcccgagtagctgggactacaggcatgcatcaccatgcctggctgttttcctcatcttctacagtaggacgtagggcagtacctgctgagacagtaagagttttcaagattaggtttacatttggtcgcatagaaccacctttttgtcatgggtcatgataaagaattgtgctagtgctcatgttttagagttgtcagtagctgtctacgttcttccattcttctaacacatttcatgctgttgtttctaggtacgtatgttgttctgtacaggcagaaggcatgcagccatttcaaaatacaattatttcttctcagtagtccccca

SEQ ID NO: 11241 - RNA, 2168 nt, Homo sapiens
  source 1..2168: mol_type = other RNA
ctgaatagctgggactacaggtgcccaccaccacgtccggctaatttttttgtattttttgtagagttgaggttttaccttgttagctaggatggtctcgagctcctgacctcgtgatccacctgatgagacctctttttaggatctgtccatcagggtagttggacttcttacatgggggcacagggctccaagagaccaaagtagaagctgccagtcctcttaaagtctagaccctgaactggcataccatcactttcactgttctcgattggtcaaggcagaggccagctcagattcaaggtcaaaggaaataaaccccaccattaatgggaaggaagtgtcaggtaatttgcaaccatctttaatctgccacattactcttccatgtgctttccattgttttgttatatttttctgttgcttgtactcctcgtttttagatgatttccaagatgaagaaggaataggaagccctattatttgccatctctaaagcctggtagtttttaaggtgtctgaagataatgggtgtggtagagacagaggcaagggcagttaattagccaagacttgatgttttcctcatcttctatacagtaacttttttttttttttttttagacatagtttcactccatcatccaggctgtagtacagtggcacagtcttgactcactgcaacctctatctcccagattcaagcagtcctcctacctcagcctcccgagtagctgggactacaggcatgcatcaccatgcctggctgttttcctcatcttctacagtaggacgtagggcagtacctgctgagacagtaagagttttcaagattaggtttacatttggtcgcatagaaccacctttttgtcatgggtcatgataaagaattgtgctagtgctcatgttttagagttgtcagtagctgtctacgttcttccattcttctaacacatttcatgctgttgtttctaggtacgtatgttgttctgtacaggcagaaggcatgcagccctaaagcgggtagggtggagaaaagatgcataatcaggccagcaaaagagggaaacagatgggttgtgggagatgaccctgcccccatgctgtttttgttctggctgctgttgatcatatgtgaatcagcagcccagaaactggagttactgatcctttgataaaaaaagaaagtatgaacttagactcagtagagttataaattacaactctaaaaagtgattcaggttttacagtaaatacaattacaggagtattcaggaattggtaaaggggacttaattatgatggctatacctcaacatttttgggtcttgtctctagattatcatagtttacgagattttatcctgtgggctctttcaaaatgaatagagagtagtgtgtttgttagagaaataaatccaatgtgtatattttatgccaaattagtcttttgtcagtgcttgtatatgacttctggtctattttctaatctcaaggttaaggaaaccttgctgtgtctcactgagtcttcccatcattctgtggaagaatcttattttttaaaaaatactaggagaatgttatcaaacatatacaaatgtagagataatagcataatgaatttctaaatacctaataaccagcttcaacattatcaacattctgcccctcttgttttgtgtgttcttcctcactccctgcctcatggccttgatggaaggattttattctatagtatagtttaatattggtgttttaaaggatgtatcctgaaacttttgaaatcccctaaattaacaaatagcactatataatttacccaataaaaatatttggtaaagtgtgtgtgtgtgtatgtgtatagatatatgtgtaaattttaagtgatctctttaagcccttaataattctgtaaatatggaacttaattacagaactattctgaatcgaacagttgctaaagcagtttttcagattgcttatttcttttattctggttagtagtaggcacaaccatggggttcaggtctgtagaatttgatattcttattttctttcttttctttttgcattgtaatatagtatcaaacagtcctttctttaaactattaaaaatgtatgtgttctgtcaggcaaggtggctcacgcttgtaatcccagcattttga

SEQ ID NO: 11242 - RNA, 1352 nt, Homo sapiens
  source 1..1352: mol_type = other RNA
ctgaatagctgggactacaggtgcccaccaccatacctggctaattttttgtatttatagtagagacggggtttcactgtgttaaccagggtggtctcgatctcctgacctcgtgatctgcctgcctcggcctcccaaagtgctgggattacaggcgtgagccaccatgcctggctgcttatcctcttattttcaaggcgaacaggcaatttcacacaagtctcattttttaaatttggggtagagatctggaccatgctggtcacaagcctccttcagagttctgtgaaaatggacagcgtcttcttgattcaagtatgttggagtgaggtcacatccaccaccaaaccaccactgcttgttgccatcagcttcttctacttcaaagtatctgtagttgaaatggatagtaggagcatgaggattcttggggtggataacagagctcacgcccatagcacaaaatggcaatttaccatctttagtcttcagaacttttcctctgcttctcatttgttttgcagcttcctctgaaagatttccatgaacaacagaaatgctcaccccagccttttcgaaaacacacccatcttgaagtacacagctgatgccgccacctccttccttcctctcccaccggtccacagaaaagttggcgcccccgtctacctgtgccagagcctggcacacctgggcctgggtctccagaatcagcagctccatcttggtcttcatgtcgcccggcctccttcgcagctcgcccaggtcggtcacaggcggggccatgaagctgctgcagcggtgggccagctcatcctcctcctcctccggcctccccagcgaagtggcccgcgtccccgaggtcttaggcaacatctccgcccgctgcacatgcccgaaggcggcggtggccagccccaccaaccccgccagcgccgcggccagccctgtccccacccaggggccgcctctcgacgtcgagccgtgccccagcccgcggctctgctccgtgccagccgggccagggggccggcagacgcgtccggctgcgctgcgctgggaccaggctcggagccctccgccgccgcactgggaccaggcgcggggccctccgcagccgccccgcgccacgagccagcaggggcccgagctcagcctgcccagctgcaaggccatgttcccgcactatcacctggagcagtgcctgcgtcccagagccctgcgtttgagccccccacccagacccccggagtattgagccggcgagctgcacaggcggaaagaacctttcgagaagagccgctgcagcgtcgggctccggaggcgggggcgggaactggggcgcgctggga

SEQ ID NO: 11243 - RNA, 6073 nt, Homo sapiens
  source 1..6073: mol_type = other RNA
ctgaatagctgggactacaggtgcccaccaccatgcccgactaattttttgtatttttagtagagaaggggtttcaccatgttagccaggatgggctcaatctcctgacctcgtgatccactcgcctcggcctcccaaagtgctgggattacaggcgtgagccaccgcgcccagccttgtttttttaatttttaaagaaaagactcgagtaagtcaggctctcagggaccctgcctgagtccccagtggaaatggttcgtcttagggctgcatcatttgccccagccaacttcttaccaactggagggtctcaaggtgggcccccagaaggtcctgcagggctgggagcccagaggacaaatatggctaatggaatccagcctggactcttacatctggcaccagttcagcaagtgaggatataaaaaaccagacatcacctcatcgctgtctcatcaaaaaaggagactttctcgctgcacattcctgcagaggacaaattcctgctcatgtattgcttgggagggagcaagaagagcagagtagggaatctgaggagttctccccttcttgggaatgggagagcagcccaggtcatcacagcagccctgagactggcctcttggtaaccatgacaacctcagctcccaggcactgtgtggacatctgacatgcggagaccctcctccactccttcctacaactctgaagaagaacctggttctgcgaggtgagggggcttgtctgaggtcactgagctgcggttggaacttgcccctgtctgacgaactcccacgccgatgctctcagcttcccaggagccaagaggcctgtggtctaagcgcagctcttctcaaactgtgtgagtgagcttgggcaggtctaagacccctcctgagtgcttcagtatccctctcaggatgtccagaggaaaactccaggctgccccacctcttcctccaggatagtctgtcatcagtttacacgttgggctttccgagaagtggaagtgttggcgttcagctgtgggtccgtctgaccttggaggtgacttctgaactattaggggactaagcctccccaagcagttactgctgattgctcaaaggcagctgctccccttcacacagagggtctatccttggaaacttgtgccagggacattctgagtaaggtagcagatttacgttcattagactttctcagaggatgcagtttgctgaacctcaggttgtctcttcatctgcagtcataaaatattcaagccagaaggcactctggtgattggaaatgctaatctctgtaatttttttttctttttttttgagacagggtctcactctgttgccaaggctgtggcgtgatcatggatcactgcagtctcaacctcctgggctcaggtgatccttctgcctccacctcccggatagctagatagctggaaccacaggtacatgtcaccatgcctagccagttttttgtatttttcgtagagacagggttttgccatgttgcccaggctggtctcaaactcctgggatcaagtgatcctcccacctcagccacccaaagtgttaggattacaggtgtgagtcaccgtgcccagcccattttctttttagagacggggcctcgctctgttgcccaggatagagcgcagtggcatgattatagctcactgcagcctcaaactcctgggctcaagtgagtatcccacctcagctctccaagtagctgggacttcaagcatgagccactgcacctggctaatttgaactttttaatttttttttattgtagagacagggtcttgttttgttgcccaggctggactcaaactcctggcttcaagcaatcctccttcctcctcagcctcccaaagttctgggattacagacatgagccaacatgcctggtctagtcttaccttttactaatgcggaaactgaagcccagagatgcagagatgtgcctaaattacagttaattaggaacaaatgtaatcctcaaatccagatctccaacattcatgtcaaaactccctaaaatcaaacaacatcggctggggaaagaacattcaaagtctcccagtccaagcctctcatttcacagtaggagaaagcttgactcagagaagagtggaatatgcctaagagtgacatgcaggcaggcagaatgcaccatcaatgaatcgaaaagttagttttttactatatgtgccctaaggcatataaagtgacttctccgagcttcacctttgaaatggaaataaaatttacagtatagggttcactgtcaggaggataaatgattcatgaaatgcccttgggccagcacccagcacttagtgggtgctcaatgcatggtatctattattaatactgctagaaccttgtcatttccccctctgccattctgccttccaggtcaaacctttctcagtacagtatagtaggtaagactggggactactgcttcagctacttgtcagcagggtgactttggactggttactacccagcaactctgggcctcaaatgtctcatcagtaaactggggacagaatagcagtacccaccagacaaggctgtgggagggggaaataatgcatgtgactggccttcacacaaagccaagcacatagtcagtgctcaataaatgcgggctactactgttaccaattacttccacagccatgtctcatgtctgtcaccatcccagactgcagggagtctggtccaccagcaagtggccggtccccaacctccagggctctccagtctcaagagtgctgacgcagcaagggaaggagctcccagtacatccacaccggctctcctgactcagctctgatttctcaggtgcctgtgtagggtcgacaattctgagcatgctggacgaaatcccgatttttgcattcatgtaagagtcttggaagagcccccttttcacacgtgcagaaactgaggtctggggaggaggaagaggctgctgcccacggacacacaggtgccaggaccaatgtctggggaggaggagaagggcgctgttcacggaaacacaggcgccagggcttgatgcaccggtgtcctcgcttgtggctgggtccttctgggacgatcccctttcccaggatcccgcccctaggaagagcaccggccatgcccctacctgagccccaccccctgagttctttgagcaccgctgcccccaggccgttacgatgagggaagccacgacagccaaggctacggctaccttcctgcagcccctggggatgccactgatgcgacgccgcggcggccaaggcggggctgaaggcggcgcgcccggcttccctgagccagtttggaggagcgctcttcaatcttccgaggccggatgaagcattcgggcgttcccactgcggaagggcggggatggctgtgacgcaggcgtgcccgccgtcgcctgcagggggcgctgttgctggcgcgattctatcaagcgcagagccagccgaggcagtatgccgaggcagagaaaccggttctgcagtcccagggcctcggtttccccctctggagagtgttcgtttgtgacagggtctcgctctgttgccgaggctggagtgccgtggcgtgatctcggctcactgcaacctccgcctctccaggtttaagcgatcctcccacctcagcctcccgaggagctgggaccacaggcgcgccaccacacccagctatttttattttattttattttttgtagaaatgaggtttttctgtgttgcctgggctggtctcgagctcttgggctcaagcgatcctctcgcttggccgcccaaagtgctgggattagaggtgtgagccactgcaccgccgaaagtgggtttgatgacaatgttgtgaggcaaagcttcttagagttgtggagcctagggccgggcgtggtagctcacgcctgtaatcccaacactttgggaggctgaggcgggtggatcacgaggtcaggagatcgagacattcctggttaacacggtgaaaccccatctctactccatcctcccagcaccacctgcaaccagccccttgccctctgcaaactggagcacgactggatctttagatgggggaaaaatgcttcatcatgttctgctgcttcatgcaaaaccagaaactccctccccctcttccctcctcccagcgcactctccttccagtaaaaagtggttaaagggacagcgccatcaatttcccagctctgagggtctgcttagaactagggggctggaaggagacagagggcaaagagaaaggaactggcagaggtctttcctgggggatatgtctgttctgtcctggggatcctggagcaggaaaacccgcgtaaagtaggggtgtagtgggtgttgagataactgcctgggggaggttcagagtggaagtacgagtctacaaactctcaagggcgtctcagggctcccagcatccccaggggtcctttcgcaggggtccctaagcaggaggggaacagcccagaaaacacggaactggacccccgacaggaagtccagggaggggtccctggctcactatgtgaccctgctggatcacttgcctcccctctcgggtcccctcagcacagtgtccctcccttccttcccctaaagtaaaagcagagggttaatctctttccccgccccacgcccaacaaagagcaggccctgtccccggtgctgaagcgccagccgcagcaccacccccactcccacagcataaaacatgagccaaaaccaataaagagccaaatgtcacagccgttgcagggccccctaaatcctggggaccccttcttctacctgacatcctattggggtgagggactttggtactcagaaagcatctcatcacttccctgtaagagagaagggatgccgactcaggcgcctgcttgtctgttacaggagtgggggaagagaggacaagttgaggctgagaagatggggagggggagggagaaaagaggacttcctagtgttgacagaacggcaagatgtgggttccccatccccagttcagccagagacccctcaaagtggaacttcctggggcagtcgggggtcaggagttggagcttgtctctggggcaagaccccttcgttgtacagatggaaaaacaagggtgggaggacacagcttgtccaaggtcattcgaccagcaaactgcctagctgaccccagtgtgcagaagctggctcgggtgacacccatcatttccccccaccccacacaggggccagctctctcaacttcatgcccaagccctcctacggtacccccactgtaggttctctgcccctcaaactcagcccagctttctcctgcctgttcaggggaccttctgcccgcttcgctgagggtccgtcccctttactggggctggcagcagggtctcccatctcctctctcgggggccactgcagactttttagagaacgccttgcctccccccaaccccacccatccggggttccctctctccatcctctgcagtgtctcccatacccccattcagggtagccttgctattctccccaactccaggtcccccttcatctattccggggctggccgcggagtttcctgagcgctctccaagtgggtcctctagatgttaggagaacactgtacctcccccggtcaggggtctcctgtctccgttctatggagcgtccatgctcccattcaggactgccttgctccctcctctgttccggggctggctgcacagtctctgcaccccctatcctgaaagcctctcttaactatttggaaagcctcgtgtcctgtctcatacagggatcccctcatcctaatgactgcaatcttccattgctccatcccgagggcatcctgcccctattcccatcaggtttctccttgtcctctccctgtttcaagtcccctttcttattccgaacacactcgcaggctcttccgacgcgcacccgggggtcctcactggcccactccgggagtcctctgcccgcttccccgacctcgagggtctcctctgacgcagcgtcgattcc

SEQ ID NO: 11244 - RNA, 3635 nt, Homo sapiens
  source 1..3635: mol_type = other RNA
ctgaatagctgggactacaggtgcccaccaccatgcccggctaactttttgtatttttagtagagactgggttccaccgtgttagccaggatggtctcgatctcctgacctcgtgatccacccgcctcggcctcccagagtgctgggattacaggcgtgagccaccgcgcccagccagatattgattgttaactctattcttcaatattcgtttagtaacaaattaagatatgttaatttgcattttaaatttgagtaaggtagaagttttcaaatatgttattacctgtacgtatttcctaatttgaaaatgaaatttagatgtcagtggtctatttgttaataagaggcaaaatgggacttcagtgctaatctaaatccaaatcctaaattttttgtaccccattctaccaaatgagatctatagaataggaatttcctctcaacatggagaagaatattctaagtctcggaactgctattgagtaatgtggcctactatgtggatgtaaattaaagtttagaatggaacctatgtttaaggagtgccagcctgtaaggctgcagaaactgctgggttccagaggggctcccaagcctgagagtctgataacacccacacatacaaacatgagataccacacaaacatacacaagaaaccgcacaaacatacatacatatttttagagtttggttcttttttaaatttcgctttgtaattttgtttgttttcctttttatttttgaatcggggtctcacttggtcacccaggcagtagtgtgattatggctcactgcagcctcaacctcctgggctcaagcattcttcccacctcagcctcccaggtagctgagactacagacgtgcaccgccacacatggctaattttaattttttttgtagagatagggtcttgctgtattgttcaggctggtctcaaactcctggactcaagtaatcttcttgcctgaagttggtctcaaactcctggccttcagcaatcctcccaccttggtctcccaaagtgctgggattatagcataagccaccgtgcctggcctcatggtaattttaacctgtaggagaatgggtgggaggatccagagggcctgagtaaagtagaactgggacaatgaagatataccaccttgatggatgccagcagaaaggtgtcttcttgggcttctgaatgtgaagaggaggagttcctcgagacaagaagagaacttctgttagctctggatccctctttatgtatctatatgtccacgcatacatttaatatttattgagtatatggcatgtgctaggcattgtatttatatacatttactggcgagcaagacatgcctaattcctccagggatcttgatttagtcattctaatggacacatgcacacaccttcataaacaggacattactgtgtgacaaatgttacaacgggaaatgcagggcactgtggaaggaaaccgatggagcatttggtgctttaccattggaaagggaggagctatctgtgaaaatgtccttgaggaagcaatttcaaagctgagacccctgcaaggattgcatttagtcactcgtagggacaggctgatcagccaatgtaaagtttatttcctcctgagcaatgggattgtgacttcaatatgtttgtgtgagtttccttggctgaagctttctcacgttacatgtcattgttcaatatcacacaactaaaacacctacaagtaaatactgactgtagcttaatgtcagacttgaggttgtaaggtaaaatcagagatgagaggagtcaaggataggatcaaagtctcttcttctagaggaatatggtcaggagagagcacaaccttagaaatttgggggggtgttgcttgaaacaggtgttgaggaagaatgcaggagttctgaggtttctgatgtgacttgggggtctgaaagttactgctgaccaggatagaaaaagatgagaagaaacttggccaggtagataagatggaagcagtcccaaggaaccatggaaggaggtgtatttccggaggtgagttagagcaaatggcatttacctggtctctgccaggctctcctctgggtgctctggtatttattgttctttttagtttttatttagtttcattttagttttagttacattgatgatgaccttcaataaagttgccttctggatagctttgatgctaccaaaaatgccagttctcagctgtaggaggagccattaaaatctaagcaagagaagttcagttttttaaagccacaactccagacataaatttgcccatattttatttaggacaggggcaaaaaatctttaagagcatgctatatactcaatactccaaattttcagtccaatttggggccttcttataggcctctagggggagttttagccccaggactcatttactggcctttttaagacctaggaacttgataatggcacggtggatctccttggtcttaatgctgtatatgattgggttaagcatgggaggcacaaaaaggtagacattggccataagaagatgaatagcaggtggggcatgcttcccaaaacggtgcaccagggacagccccatcatgggcacaaagaatactagcacagcacagagaggagcggtgcatgtctgaaaggcacggcgctgctcctcttgggaggccaggcctgctactgtgtgcaggatgagtccataggacagtgcgatgagcaccaggtccagcatcacagtgaaaactaccaccatcagtccatacagattattgaaggtgatatctgtgcaggccagctgtatcacttcctggtgcaggcaaaatgagtgggagaggaccacagatccacagtagggaaaagccttcaggaggaggacaatagggatagtggccacaggtccccggaagatgacaattaggcctgctctgaccacttgctggccagtgataatgaccgaatacctcagagggtggcagatggccacaaggcggtcaaaggacatcatgaggagcactgaggactccatgaaggaaaaagagtggatgcagaacatctggatttgacacgctccaaagtagatactatgggagttaaaccagaagatccccatagtggtgggcaacgtggacacacacagccccaggtcagtgagggccagcaaggatagtagatagtacatgggtgtgtgcagacgagggttggtcttaataatgatcagaatgaaacaattgcctgagatggcaaccatgtacataaagaaaaaggggatgaaaatccagtgtttgatgccttccaatccaggaaagctggtgagatagaatatggggctaaactgagtaatgttggatagcagcatgaattgaggactgagcgaatattggactgacattcctcggggattgagctcttatcctgattctttgtgcctggggttctgttgtcagctctgtgttcaccaacttcagagtgatgagatggacagggagaaggatctggtagaaacaagatgtcagcaggtaataacaaaaatgtgaagccaatgagtaggttccaaaggaagaaagaagagtatagataaggatgacacaagggtcactgagaggcacaaggctgtgg

SEQ ID NO: 11245 - RNA, 4001 nt, Homo sapiens
  source 1..4001: mol_type = other RNA
ctgaatagctgggactacaggtgcccaccaccatgcctagctttttgtattttcagtagagacggggtttcaccgtattagccaggatggtctcgatctcctgacctcatgatccgcctgcctcggcctcccaaagtgctgggattacaggcgtgagccaccacacccagccaattcaaaatcgtttattacttaacacccctgtcagagtcagtatcctgttatctaactcatgacgagctttgcaacaaaacatgtgaagagccctactacatgtgagaaataatgctcaagtcagcttttgctgccaagtgagctgtcaagatagatttcttaagtatgggattttggaagtgtggacaaggagctgtggatatgtattagcatacggagattggtgaaacatctccatactaacatgggtttcccacaatccagaaagttaagaattactgatttaataaattagtttaaataatttattttttcattgtagctatcattaatgaagcatttactttgtgtcaacccctgtgctgagctctttaaatatgtatgtaaaacaattatttgtcccattttataggtgaggaaactatggtttagaaagaggcttagcatatctttgaactggtaactgactaagctggacccagactgaagctgcctcacgataaaaagccatgctcttacttcatattgcacaaggtcaaaattctttagtcttcccagtttctttgtgatgttgattctaagaaaagtttctgtaattcaagtgaatgtgaaaatcctcaggctacaagatctcttttgtaaaaaacaggctggctatatgtagtcaacatttaactgatatttgtataatggaataatgtattttctcagctacaccaatattttaaatgtttgtaatgagagatcaagtgatttcagataattaaaaaaaatacagtcacactaacttgccctgatttcctttgtagaaccatgatctgcggaatcaaggtctgctgttacctgatagatgagaataggaatagaagaggccatcaaaaggcactaattataaataatatgtagatttttaacttatccttttcaagaacactttagctgtctgaatttttttaaagccagatagaagttggtaaaatgtatctgtgatgaccaaattttgaaactcctttggaattaccaaatatagcagaggtagttggcattaaggagtcacttgtatagaaacaataaagctctattttaaaaatctatgcatagggctacagcttcacctgaagacagtgttttggaccataccacactcatgggaaagcctccaattttgaaatgtagagtagcaaaaacacaacagacagtcatttcatggtacaaagcagatactataaacatgagaattaagaaatgaaaataacatatacactaaaaacatcacaacagaaacaggctttatttcaaccagacaagtgaattcttcaattaacatcaacttcttcaagacttgaagatatggaaattaaagacggtgctcagaaggcagagaaaggaagattcatcatggagtaattgttctgtccttcaaaaatccctttcaacaataagctcaatacacaagatcatgggatctcatgcatcccaatatttgtacatgaccctcatttgaaagttacccatcagtcttaatgaaatctttcaaaaagaaaaaatatatagatcagtataaattatttttaattttagaaactgagattgaagtacagtttttagtttaaaatattaaaaatgaaaaaacctttaacattattaaagatgtgttgttacaaagttcctagatatatacatgtacaaaacaaatagatattactatctgacacctcaacccatgacttaccctaaatctcctgatatgaacaattaatctactgggaggcttttcccaataagtttcaaatttcttgcacaaagatttgctgccattcatattctgtgcatggatgaggacatttaatcacagactatttcaacttaatataacctagcataaaataaatccaatgaaacactacatttataagcgataggacaaacttgcatataatttgcaacttttgccagactcattaaattcattaacacattcagtcttctcttcacgggcattttcaagagctttagatcttgtgcttaactttgtattgagctggtcagcaccttcattgatatgaacaattatgtcaaagaaaggttacaggtagggggagggacatcatctgaggacagaaacagagggaacgactcttttttcagaagacaactaaaacagaaaaacaagacaaaaaagggtacaaaacaaataacaaaagtgttcacagtaaaacatgccagatttgtagtttcatttgaaaccaacagcaaatcatgaaacgtcatgaaaaatataagtcaaggtaaaatctcctagagtaattactaaatgaagttaaaatcaccacactgatcagtaaaccccagaagaaaaatgaccagcgcttacatatcaggtccttcttaaacatcaaacaacttttcaaagttaatgcatacaattggtaggtttggccacgctgcaccatttttttaaaaaaatacagtatacagaaaaaaaaccttttatattcccccgttttgaatcattagctcaaaacctaagagtaaaagatcatctggaaggattttaaattatttacaaatccagcaggttcatctgccataatggcttggcttccgtcccaaagcgactttcaccttctccagcagcaattttttagttctctgtccttttgggaggctgtttcctccactgctcgtctctacttgtcatcagtcattttgaacagttccaacagtgccccaacggctccaaaataaccctcatgttccaaaaacagagctttcagttgtcctttggaccaaaaatccatggcatatgccagcagcttcatggagaccatattgattctgagaaaatttccaacaaacacaactctgtctatgttctcattcaacgcgcacatccgagcaatggagccaatgttgttggtgatggtgaccaatgtggcccgggcgaggtcttccttgctgatggaatctcgcttttctttactcatcatgttgccaaagctggtccctgtaactcttttatagttgtccttggagtacacggctagaatgctgacacctgagcccatgttaaccagcaacatagggtatgggttatcaaggcagtacggctttttttgacacaattcaggatttgtgggattttcaaaatagtaacattctggcttgccgttgaagccaacagagtcgacataaagcaggccctgaatcagacagtccagttcatccagtttatgcagctgcaggtcagcaatcattctgaagtcctcttcgaatttgaaagccccgcctcctgtggcacagagggtggtgtgaaggctagagaagttcttctcgctgcccatctgaatgaacctgtgcatagcacagctgggaaagcggatgaagtgcaggttccctttgcgtccacacatggtcaggtttttcagttccaggtggacgtctcggatcccagttttcccataagcagtattagaagtcaaatacttccggatgctcttcaggttctccacttcctcttgctcctcttcggctgtaatatccttcggctcgaaatacaccaatttaaccagcgttccaccgatgtccatgccaaaccatgggaatgtttgctttttgccatttataagcttcattaaagacacccacaaagaagtaaccagttgaatgagcttcagtcaagaaaaaccagctgtaaactcgacctacaaatttacatcccacagcgtcctgtggggaaggtacactttacaaactaccattatatatacaagctttagattgtgaaataatgcacttcggctttctccggtgtacattacaattac

SEQ ID NO: 11246 - RNA, 4931 nt, Homo sapiens
  source 1..4931: mol_type = other RNA
ctgaatagctgggactacaggtgcccaccaccatgcctagctttttgtattttcagtagagacggggtttcaccgtattagccaggatggtctcgatctcctgacctcatgatccgcctgcctcggcctcccaaagtgctgggattacaggcgtgagccaccacacccagccaattcaaaatcgtttattacttaacacccctgtcagagtcagtatcctgttatctaactcatgacgagctttgcaacaaaacatgtgaagagccctactacatgtgagaaataatgctcaagtcagcttttgctgccaagtgagctgtcaagatagatttcttaagtatgggattttggaagtgtggacaaggagctgtggatatgtattagcatacggagattggtgaaacatctccatactaacatgggtttcccacaatccagaaagttaagaattactgatttaataaattagtttaaataatttattttttcattgtagctatcattaatgaagcatttactttgtgtcaacccctgtgctgagctctttaaatatgtatgtaaaacaattatttgtcccattttataggtgaggaaactatggtttagaaagaggcttagcatatctttgaactggtaactgactaagctggacccagactgaagctgcctcacgataaaaagccatgctcttacttcatattgcacaaggtcaaaattctttagtcttcccagtttctttgtgatgttgattctaagaaaagtttctgtaattcaagtgaatgtgaaaatcctcaggctacaagatctcttttgtaaaaaacaggctggctatatgtagtcaacatttaactgatatttgtataatggaataatgtattttctcagctacaccaatattttaaatgtttgtaatgagagatcaagtgatttcagataattaaaaaaaatacagtcacactaacttgccctgatttcctttgtagaaccatgatctgcggaatcaaggtctgctgttacctgatagatgagaataggaatagaagaggccatcaaaaggcactaattataaataatatgtagatttttaacttatccttttcaagaacactttagctgtctgaatttttttaaagccagatagaagttggtaaaatgtatctgtgatgaccaaattttgaaactcctttggaattaccaaatatagcagaggtagttggcattaaggagtcacttgtatagaaacaataaagctctattttaaaaatctatgcatagggctacagcttcacctgaagacagtgttttggaccataccacactcatgggaaagcctccaattttgaaatgtagagtagcaaaaacacaacagacagtcatttcatggtacaaagcagatactataaacatgagaattaagaaatgaaaataacatatacactaaaaacatcacaacagaaacaggctttatttcaaccagacaagtgaattcttcaattaacatcaacttcttcaagacttgaagatatggaaattaaagacggtgctcagaaggcagagaaaggaagattcatcatggagtaattgttctgtccttcaaaaatccctttcaacaataagctcaatacacaagatcatgggatctcatgcatcccaatatttgtacatgaccctcatttgaaagttacccatcagtcttaatgaaatctttcaaaaagaaaaaatatatagatcagtataaattatttttaattttagaaactgagattgaagtacagtttttagtttaaaatattaaaaatgaaaaaacctttaacattattaaagatgtgttgttacaaagttcctagatatatacatgtacaaaacaaatagatattactatctgacacctcaacccatgacttaccctaaatctcctgatatgaacaattaatctactgggaggcttttcccaataagtttcaaatttcttgcacaaagatttgctgccattcatattctgtgcatggatgaggacatttaatcacagactatttcaacttaatataacctagcataaaataaatccaatgaaacactacatttataagcgataggacaaacttgcatataatttgcaacttttgccagactcattaaattcattaacacattcagtcttctcttcacgggcattttcaagagctttagatcttgtgcttaactttgtattgagctggtcagcaccttcattgatatgaacaattatgtcaaagaaaggttacaggtagggggagggacatcatctgaggacagaaacagagggaacgactcttttttcagaagacaactaaaacagaaaaacaagacaaaaaagggtacaaaacaaataacaaaagtgttcacagtaaaacatgccagatttgtagtttcatttgaaaccaacagcaaatcatgaaacgtcatgaaaaatataagtcaaggtaaaatctcctagagtaattactaaatgaagttaaaatcaccacactgatcagtaaaccccagaagaaaaatgaccagcgcttacatatcaggtccttcttaaacatcaaacaacttttcaaagttaatgcatacaattggtaggtttggccacgctgcaccatttttttaaaaaaatacagtatacagaaaaaaaaccttttatattcccccgttttgaatcattagctcaaaacctaagagtaaaagatcatctggaaggattttaaattatttacaaatccagcaggttcatctgccataatggcttggcttccgtcccaaagcgactttcaccttctccagcagcaattttttagttctctgtccttttgggaggctgtttcctccactgctcgtctctacttgtcatcagtcattttgaacagttccaacagtgccccaacggctccaaaataaccctcatgttccaaaaacagagctttcagttgtcctttggaccaaaaatccatggcatatgccagcagcttcatggagaccatattgattctgagaaaatttccaacaaacacaactctgtctatgttctcattcaacgcgcacatccgagcaatggagccaatgttgttggtgatggtgaccaatgtggcccgggcgaggtcttccttgctgatggaatctcgcttttctttactcatcatgttgccaaagcttgatgctacagcagatccttgaaggccaaatcgttcatagtctcctccgtaaatgtccttcaccagtttatcaacattggtgctgtcgcctttagctgccatttccagagcttcttcaaaggtctcacaaccagtcagcaagcaacataggcctaggaatgttccacctccaagactggtccctgtaactcttttatagttgtccttggagtacacggctagaatgctgacacctgagcccatgttaaccagcaacatagggtatgggttatcaaggcagtacggctttttttgacacaattcaggatttgtgggattttcaaaatagtaacattctggcttgccgttgaagccaacagagtcgacataaagcaggccctgaatcagacagtccagttcatccagtttatgcagctgcaggtcagcaatcattctgaagtcctcttcgaatttgaaagccccgcctcctgtggcacagagggtggtgtgaaggctagagaagttcttctcgctgcccatctgaatgaacctgtgcatagcacagctgggaaagcggatgaagtgcaggttccctttgcgtccacacatggtcaggtttttcagttccaggtggacgtctcggatcccagttttcccataagcagtattagaagtcaaatacttccggatgctcttcaggttctccacttcctcttgctcctcttcggctgtaatatccttcggctcgaaatacaccaatttaaccagcgttccaccgatgtccatgccaaaccatgggaatggcggcctgttctttctccccgagtccatcctcctccgcagccggcatttcttggccggggagtcatgctgagggagcagtggctgcggctgcagctccggcaggagcgggaggcgctggggcgccgcgtcgctgccgcccactggaccccggctgcagacgtgcggcggctggactggcggcggatggaagccgttgtgcagcagcccgttcacagcggcggcgctggtgcccacgggggcccctggagagtgcgggaccgagcgctcctgctgcccgctgcggtcgcccatgccgggggctggcggggctgtgcgcgggccccggctcaggcggcctcgctggaggtcattctccggcgtctttatttccccggatcctccctgcggcttccgattcagcagccgcagagccggcgcctggggatggcgaacccggcgctcctcccctcctcctgccgactcccccacctcctctgcgccctgccccccgcgcgccggccccacggcgccggcctggagcacgccagccccgggcgcggaatcggggatccccgcgcacccccagccggggctcccgccgcccgccttcccctgatccccaggccgcgcgacttcaaacgcggcttcctcgcctcccagactggtccccgccactgagcatgcccagtcctgcccgccaccgccaccgacgagtttcaacatggggaatcaagttctctgggcttgcagagaggagatgggcgggttgggctttgtatggcgatgtgaaaaccagatgggtctgggagagacagcgaaaggagcgaaccgtttcaggaggaatacgggaggaagacaattatttgcagaggtgtcaggtttgctaatcctgtccccagtgagcaagatacctttgcaaggtcattcacgttaccctccccgctttgtgagtgtgtgcttacgcgcgcgcgcgtgtgtgcctgtgcgtttggt

SEQ ID NO: 11247 - RNA, 4178 nt, Homo sapiens
  source 1..4178: mol_type = other RNA
ctgaatagctgggactacaggtgcccaccaccatgcctagctttttgtattttcagtagagacggggtttcaccgtattagccaggatggtctcgatctcctgacctcatgatccgcctgcctcggcctcccaaagtgctgggattacaggcgtgagccaccacacccagccaattcaaaatcgtttattacttaacacccctgtcagagtcagtatcctgttatctaactcatgacgagctttgcaacaaaacatgtgaagagccctactacatgtgagaaataatgctcaagtcagcttttgctgccaagtgagctgtcaagatagatttcttaagtatgggattttggaagtgtggacaaggagctgtggatatgtattagcatacggagattggtgaaacatctccatactaacatgggtttcccacaatccagaaagttaagaattactgatttaataaattagtttaaataatttattttttcattgtagctatcattaatgaagcatttactttgtgtcaacccctgtgctgagctctttaaatatgtatgtaaaacaattatttgtcccattttataggtgaggaaactatggtttagaaagaggcttagcatatctttgaactggtaactgactaagctggacccagactgaagctgcctcacgataaaaagccatgctcttacttcatattgcacaaggtcaaaattctttagtcttcccagtttctttgtgatgttgattctaagaaaagtttctgtaattcaagtgaatgtgaaaatcctcaggctacaagatctcttttgtaaaaaacaggctggctatatgtagtcaacatttaactgatatttgtataatggaataatgtattttctcagctacaccaatattttaaatgtttgtaatgagagatcaagtgatttcagataattaaaaaaaatacagtcacactaacttgccctgatttcctttgtagaaccatgatctgcggaatcaaggtctgctgttacctgatagatgagaataggaatagaagaggccatcaaaaggcactaattataaataatatgtagatttttaacttatccttttcaagaacactttagctgtctgaatttttttaaagccagatagaagttggtaaaatgtatctgtgatgaccaaattttgaaactcctttggaattaccaaatatagcagaggtagttggcattaaggagtcacttgtatagaaacaataaagctctattttaaaaatctatgcatagggctacagcttcacctgaagacagtgttttggaccataccacactcatgggaaagcctccaattttgaaatgtagagtagcaaaaacacaacagacagtcatttcatggtacaaagcagatactataaacatgagaattaagaaatgaaaataacatatacactaaaaacatcacaacagaaacaggctttatttcaaccagacaagtgaattcttcaattaacatcaacttcttcaagacttgaagatatggaaattaaagacggtgctcagaaggcagagaaaggaagattcatcatggagtaattgttctgtccttcaaaaatccctttcaacaataagctcaatacacaagatcatgggatctcatgcatcccaatatttgtacatgaccctcatttgaaagttacccatcagtcttaatgaaatctttcaaaaagaaaaaatatatagatcagtataaattatttttaattttagaaactgagattgaagtacagtttttagtttaaaatattaaaaatgaaaaaacctttaacattattaaagatgtgttgttacaaagttcctagatatatacatgtacaaaacaaatagatattactatctgacacctcaacccatgacttaccctaaatctcctgatatgaacaattaatctactgggaggcttttcccaataagtttcaaatttcttgcacaaagatttgctgccattcatattctgtgcatggatgaggacatttaatcacagactatttcaacttaatataacctagcataaaataaatccaatgaaacactacatttataagcgataggacaaacttgcatataatttgcaacttttgccagactcattaaattcattaacacattcagtcttctcttcacgggcattttcaagagctttagatcttgtgcttaactttgtattgagctggtcagcaccttcattgatatgaacaattatgtcaaagaaaggttacaggtagggggagggacatcatctgaggacagaaacagagggaacgactcttttttcagaagacaactaaaacagaaaaacaagacaaaaaagggtacaaaacaaataacaaaagtgttcacagtaaaacatgccagatttgtagtttcatttgaaaccaacagcaaatcatgaaacgtcatgaaaaatataagtcaaggtaaaatctcctagagtaattactaaatgaagttaaaatcaccacactgatcagtaaaccccagaagaaaaatgaccagcgcttacatatcaggtccttcttaaacatcaaacaacttttcaaagttaatgcatacaattggtaggtttggccacgctgcaccatttttttaaaaaaatacagtatacagaaaaaaaaccttttatattcccccgttttgaatcattagctcaaaacctaagagtaaaagatcatctggaaggattttaaattatttacaaatccagcaggttcatctgccataatggcttggcttccgtcccaaagcgactttcaccttctccagcagcaattttttagttctctgtccttttgggaggctgtttcctccactgctcgtctctacttgtcatcagtcattttgaacagttccaacagtgccccaacggctccaaaataaccctcatgttccaaaaacagagctttcagttgtcctttggaccaaaaatccatggcatatgccagcagcttcatggagaccatattgattctgagaaaatttccaacaaacacaactctgtctatgttctcattcaacgcgcacatccgagcaatggagccaatgttgttggtgatggtgaccaatgtggcccgggcgaggtcttccttgctgatggaatctcgcttttctttactcatcatgttgccaaagcttgatgctacagcagatccttgaaggccaaatcgttcatagtctcctccgtaaatgtccttcaccagtttatcaacattggtgctgtcgcctttagctgccatttccagagcttcttcaaaggtctcacaaccagtcagcaagcaacataggcctaggaatgttccacctccaagactggtccctgtaactcttttatagttgtccttggagtacacggctagaatgctgacacctgagcccatgttaaccagcaacatagggtatgggttatcaaggcagtacggctttttttgacacaattcaggatttgtgggattttcaaaatagtaacattctggcttgccgttgaagccaacagagtcgacataaagcaggccctgaatcagacagtccagttcatccagtttatgcagctgcaggtcagcaatcattctgaagtcctcttcgaatttgaaagccccgcctcctgtggcacagagggtggtgtgaaggctagagaagttcttctcgctgcccatctgaatgaacctgtgcatagcacagctgggaaagcggatgaagtgcaggttccctttgcgtccacacatggtcaggtttttcagttccaggtggacgtctcggatcccagttttcccataagcagtattagaagtcaaatacttccggatgctcttcaggttctccacttcctcttgctcctcttcggctgtaatatccttcggctcgaaatacaccaatttaaccagcgttccaccgatgtccatgccaaaccatgggaatgtttgctttttgccatttataagcttcattaaagacacccacaaagaagtaaccagttgaatgagcttcagtcaagaaaaaccagctgtaaactcgacctacaaatttacatcccacagcgtcctgtggggaaggtacactttacaaactaccattatatatacaagctttagattgtgaaataatgcacttcggctttctccggtgtacattacaattac

SEQ ID NO: 11248 - RNA, 1159 nt, Homo sapiens
  source 1..1159: mol_type = other RNA
ctgaatagctgggactacaggtgcccaccaccatgcctggctaattttttgtattttagtaaagagggggtttcactatgtttcccagggtggtatcaaactcctgagctcaggcaatccacccacctcagcctctcaaagtgctgggattacaggcgtgagtcaccgtgcccggccagattctgcatttctaacaagccccaggtcataccaatgctgctggtccacagaccacactcttgagtaggaagagtatggactgtgtccactgcactcacggcccctcctctgcccccaaacagaaggcaatgtgaacaggagcagttacttgacctccttgattggaaggaagcacatccgcctgggggcaggctggccttggaggatgtagggagggcagggagaagacctggaaggtctctacttagctggctggagattagaatcaggagcccagggttgggcctgtgcctcttccccacctccttcgatgtgaatagggccaggggcggcagtgtgcggaggcccctctgcttgcaatccgggtagcgctgatagcgggccagatttacagcatacatgttggagatggagccaccagggcagaagattccgtccccagagctccagcccaccagggcccgcagtttcctcagcacctcctcttccatgagcacaaacacgggggcgatttcatatgtgtactggctggtgttgaggctctcagtgataatgcgcccggccagagcatggggatccaacccagagaagagctggttgaagaaccgagggtgaccagtcttgacactgtagcgaatcacagcccgacaccgctccaggatctgcttctgtgactcgccctggctccgcagctccaaatccagcagctgcttcagctcctcaggctccttccactcacagaccttctgggagacactggttcctttctgaatggcctcatccacaacaaccccaaacacggcccggagcaaggcttccacagccactgggtccccagcaagggaggggagtgcttctgagtcagccatcaggatctctctgctcaggagagccggaggcagggtgcacaggtagctcccgctctgaggctgcccccgctagtctagctgccgagcccggaagtggatgcagccgctcg

SEQ ID NO: 11249 - RNA, 4270 nt, Homo sapiens
  source 1..4270: mol_type = other RNA
ctgaatagctgggactacaggtgcccaccaccatgcgaagctgatttttagtagagacagggtttcaccatgttggccaggctggtcttgaactcctgaccccaggtaatccacccaccttggccccccaaagttctggaattacaggcatgagccactgcgccaggccgaaataccagatcttcatggcagttgtcttagaggtagagaagaaaacagccagactgagccgggtgtggtggctcatgcctgtaatcccagcactttgggaggctgaggccggcagatcagttgaggttgggagtttgagaccagcctggccaacgtagtgaaaccccgtctccactaaaaatacaaaaattagccaggcatggtggcgggcacctataatcccagctacatgggaggctgaggcaggagaatcgcttgaacctggaaggtggaggttgcagtgagctgagattgcgccactgcactccagcctgggtgacagattgagactccatctcaaaaacaaacaaacaaacaaaaaaaaccagcctgactgaattcagtcacagtaattatacatgagtggttgctagttcctttaaccacaccagaagcattttaaagggaagatgtttcctaactccagtgattttcatgggctgaattccaggcagttcagcaaactcaacaattccggtggtatgagaaagggcattttggagtaggagatttcggctctgcctaggaagatacctcagaaaattcccctcgtgcaatttcactttgcatatgcttctcctgttcttccatttctaatccataaaatcccaaaatgcttgggagggtttattttgattttttttaacaatactgccctgctggcaacagccacgatagtcacttgctcatctgaaaatgccttgcactttctttttcactagcttcgtgtatgacgcaaaacagaaatatttcaattacaggtgactaagagtaagaaaaatatacaactatatttaaaatacttaaattaacaagatagtacttttccattctaacaaaatatcatacattcagtttaaacaagagttaatatccagacacacgttttcaaaatacctgatgctagttgaaaattagtgaccatgaggctttccaagatatttctaattagcaaactgtgtacaattttgaagaagtgtacacaccgtgctggaagacagacactgaacaggtcaaaatgcaaactcatgtatctttcatcaacctaaatcttgttgcttcacttttctaaatgatactttggctgtcagcgaatcttatagcttcttttcccttaaagacaataatatataacaacaccaccccacacaaataaccataaacttctttgtgtgaaataagccctatcaaaatgtgttcatgtatttctgtaccaactgatctatactgagactgtcatgaaaaaggtatcaaacaagtgtaacaggcctacacttaaacctctgcctcaaaggagaaatcagatacttgccacgttattgcaaagtcaaagctgctacacttaaaatatggtagatagtttagaaaaatcaaatcaaaaatgttttctcactggctttttcagataaagaagttggaccacaaaccaacacatctgtgtgaaaacagccaccaatttgagtccccccagcccctcaaaaaggaacaatgccaccagtccctcacaatgaccataacgtctctggccaggactgcgatttctagcgcgtgtcttcacattctatctctggggaagcaagacaaacaggctctacccatttccctccttttgtctccacaagccagcacctaagatcctctgaatttgttcccatccaatcctgcaaacttccaagaagggcagtagataacttttcaaaagaaaaagaaattgcataaggtccctacataatactgaggctgaaacgagaagaggctgtccactgtaaaagcaaggcacttggggcaggagccaggcaggtggcctgagcagggtccctctcagtgagtcaacagtttgaggcgcgtaaaccagctgaccaggagggacggttctgtggacgaggacttcgtagctgaggagccagatttctttttggtcccttcctcctggaatggaatcgtggcgctgctgtggagatctgagttgatgtagcacctgcttcctcggatgtagtccgcaccccggaccagatgccgctcggtcgtgggtctggagaaccggtatgggggagaggagctctcttcaatgatcggaggaatccgctcgttactgaaataccggcaaagggcatcctcccctttcctgccatgacctcgaggtctggcaaaagggtccacaatccccatccagttcccatcagcaggcatggacaaaggccgtggcttgccataagatggtgttttctctctcatttttgtgggcagaatgttggtttccaccgagtacccaggcaactgatccgagtctgcaatggtgaatcttcgtctccggctttcctggtccaagaaggaattcggggactctgaacccttaggaccaggcaatggttgtttgcacttactggaccctccataaacaaaactgccattctcatcccggggagagtagggaacagcaggcggaggaggaatataaagatccaggatggctgacttctccttcttcagtgaggtatccatagtgctttcaggggactgggttgtcgcgggtggaggtgaggtctgtacaagaggtggcttccaccgtaggtttttcaggggagcaggagtaaagttgaaagacccggtggggcgcttcttaagcagtaacacaactccggtgggattctctctcaatttcttcaccagatttttcagctgccatcccaccacagtttgctgattaacttgaatgacttcgtcaccagcatgaatcttctgagatctgtctgcaggagaattttctgtggttccagtaatcacgtgtaacccatcataggttgatttgatgtacatgcccaggccttccccaggtttaatgtttggtaagtgaacttcctccagacatgcacactggctcatcacaggatctgtggtagatcggattgttttgtcacagatgccatttaaaaccttgaccacagttaaaactttatcctccatttccgctacaaagcaatccttctggactgtagtggtcaggtccaagcaaagctggataattttgttcttcgtgactgagaaatcagtgatccctgtaaacggagcccggtccagccacgccagcagggccttggcggcgccgatgagctccaccaccgaggtcaggaactcattgggggccttgcgggaggtgttgccatcgtaagcgggacttttccgtcggctacttatgtaattctgtaaattgtgggaagatgctctcagtttcagaaccaagttcttcatgttatcagtttcgaggccataattcagtgcacagagaaggtccacagcctccaacacaagctcctggtgtccaatccgtgtgacccccagctcctccaggtcctgatgggaaatctgcagcagctgctcgccgttgatcttctctcgttcaaacttgtggacatattgttgcaggcagtcatccaaccctctagtccagtccaccacttgtttggggctccacttggtcacgggttccatggtaaaccgcttcgcctctcgctgggctggagagtcgcagataaagtgctgctgcctgcgctccggtgccccttcccgggagggcgcgcccgcggctgctcccctgcgcccgagcgactccgtcaagactgcatggccgcggtcagccagtcgtcccagcgcggctccgccaggggagcccggccctctccctccagctgccacagtccagctgcagctcctccttcccccgccgccgccgggatcccgggcacagctgctgctcccgagcgacggcagctgcaggcacgccgggctgcgaccccagacccctggcctcggctcggcacgggagcctcccggcccgcgaccacttcctcggatctctcgaggcgcgatcggctctccctcggccggtcttctcgcctgctggctctccggggtccccgctccgcgtgcgctggcgtcccggagccttcccggcgcaggtcccacctcctgcgccgccctcccgtgccgccctggcagggccgagcgcagagcgtgcgcgctcgggttgcaaagtttcagctccggttgctgcaaaccgaat

SEQ ID NO: 11250 - RNA, 1083 nt, Homo sapiens
  source 1..1083: mol_type = other RNA
ctgaatagctgggactacaggtgcccaccaccatgtccagctaatttttttgaatttttagtagaaactgggtttcaccacgttggccaggatggtcttgaactcctgacctcaggtgatccacctacctcggcctcccaaagtgctgggattacaggtgtgagccaccacgcccagcctctcactggttttagtatcatccctgtgcagcacgaaaaatcctcttggctttgtaggtctaccagagacatccctcctggcacctttcatccaccacatccagttttggctggctgcactttggacttgctgtgtggtgttctctttgggaatttttgtcatctcctttctgtgctgaatgacttgtttcccagatcccatgggttttcttttttgtggaccattccctagctctggggagcatatctgcctcaaattgattgaagtagaggtgcagaagtaagccagaaatcctttactgctgcagtaacagcagcagtagctgcaaggtttaaaccttgccgtccaaagtttaccatggtttcatagcctcgttcctttgcttgtacaatataatcatcaatctccctttcctttgaagaaagaagtggatgaaggaattttctatatattaaacttgctcctttggtatagggagaaagcagccatatgacaaaagcaatcttcagctcatagtacaggggaaaccaagcaactgtttgatcggctactgtttcaatcacagtatagagagcaaaaacaatccagtacatcatccatcgaacatattccttcacgttttttgttttcacagctttgtatgaataatatgcaggataaagcattccaaacaccagcaccacggctctggagatcatccaggacaccatcttcacgggggcttgggccccacgtccggggcgggtgggcgcagggcgctgcggaccaggccgccaacggcaggccgcgcgcttcgccggctcctcgcgctccccggggccgcgctggcgccctcaggagccgggcccggtgtgtgcgcgcggcggcctgggctgcgcagaggtcggtcccccgcccgtcccc

SEQ ID NO: 11251 - RNA, 2756 nt, Homo sapiens
  source 1..2756: mol_type = other RNA
ctgaatagctgggactacaggtgcccaccaccatgtccagctaatttttttgaatttttagtagaaactgggtttcaccacgttggccaggatggtcttgaactcctgacctcaggtgatccacctacctcggcctcccaaagtgctgggattacaggtgtgagccaccacgcccagcctctcactggttttagtatcatccctgtgcagcacgaaaaatcctcttggctttgtaggtctaccagagacatccctcctggcacctttcatccaccacatccagttttggctggctgcactttggacttgctgtgtggtgttctctttgggaatttttgtcatctcctttctgtgctgaatgacttgtttcccagatcccatgggttttcttttttgtggaccattccctagctctggggagcatatctgcctggacaaaagataaccagtaggtaaatcttgtgactctgcatgcctagaattaagaaatttcttaattctaagctaacacaattgagagcttgactgttaatagttcttgagggtgaaaatcatgatggtatcatggatggtattactgtcttcaagctttcactgtcactgtttagaaatttaatgtcattctgattctacatcatttaaatgtgacatgctttttttttgagatggagtctcgctctgtcacccaggctggagtatagtggtgtgatcttggctcagtgcagcctccgcctcccgggttcaagcaattctcctgcctcagcctcccgagtagctgggattacaggcgcccccccaccacgcccagctaatctttgtatttttagtagagacggggtttcaccatgttggccaggctggtctgaattcctgaccttaagtgatccatctgcctcggcctcccaaagtgctgggattacatgtgtgagccactgtgcctggccaaatgtgacatgctttttatatttggaatctttatgaattctttccttatcactggtgttttgggatacccaatgacttcacttagagtcagtcattcttttcattcattgtgctaagtacttggtgggtcctttcaatctgaagattcatatccttcagttctgggaaatattattgtattatttctttgataattgcatctattccctctttttagaattcccagtggctggattatctcctggataatcttttttagcagatatggaaatcaggaatgcattttcactaagcaagaaataaaaaacaaaatgaacttctaaaataaaacatagtcctttaagctgaaaactttgctatttctgtattcatttataaacctatcctaataaaagaaaaagcctttaaaagccaaataacaagaaaactatgctatattaaagtgctgaccattaataatcattaataatatagttatcttacatgtatagtgctgcatagttaataaacttccatttaaccctcaatgtaatgctattaggtatataatttgaattttccttcttgttcattacattcattttgatacttgagtcaaagacctctctgaaaagtgaaagtgccctcatttcatatcccttcactattagttatataaaatcaccactcaactggaatatttatttccatagagttgttttagttcaagataactaaaacagactaacttgaaagcagaatactattcaatctcaatttaatttaatagcaaaaaacttaaattttcacttgaattttgaatggagatagacacatgatatttatgtttattgggctcctactatatgcaagcaagcactgtgcttttaaatattctcacaggtatattacccccattttatacatgaagcaactaaggaacacagaaggctattttctttccataccaaacacaccaaaatcaattatgctaaagtatttaaaataaatcacacaaattacaacatgcaaagaaatccaaaaccataatgcaaatttttacagaacacattcatttgataacttggcttgcaaacacaacaaatgacattagtaactggctaagtaccaagttttaagaacagactttttcatgccttattttgaataatcggttacctcaaattgattgaagtagaggtgcagaagtaagccagaaatcctttactgctgcagtaacagcagcagtagctgcaaggtttaaaccttgccgtccaaagtttaccatggtttcatagcctcgttcctttgcttgtacaatataatcatcaatctccctttcctttgaagaaagaagtggatgaaggaattttctatatattaaacttgctcctttggtatagggagaaagcagccatatgacaaaagcaatcttcagctcatagtacaggggaaaccaagcaactgtttgatcggctactgtttcaatcacagtatagagagcaaaaacaatccagtacatcatccatcgaacatattccttcacgttttttgttttcacagctttgtatgaataatatgcaggataaagcattccaaacaccagcaccacggctctggagatcatccaggacaccatcttcacgggggcttgggccccacgtccggggcgggtgggcgcagggcgctgcggaccaggccgccaacggcaggccgcgcgcttcgccggctcctcgcgctccccggggccgcgctggcgccctcaggagccgggcccggtgtgtgcgcgcggcggcctgggctgcgcagaggtcggtcccccgcccgtcccc

SEQ ID NO: 11252 - RNA, 150 nt, Homo sapiens
  source 1..150: mol_type = other RNA
ctgaatagctgggactacaggtgcccaccatcacgcccggctaattttttgtatttttagtagagacggggtttcaccatgttagccaggatggtctggatctcctgacctcgtgatccacccgtctcagcctcccaaagtgctgggatt

SEQ ID NO: 11253 - RNA, 2817 nt, Homo sapiens
  source 1..2817: mol_type = other RNA
ctgaatagctgggactacaggtgcccacgaccacgcctggctaattttttgtatttttagtagagacagggtttcaccatgttacccagaatggtctcgatctcctgaccccatgatctccacccgccccggcctcccaaagtgctgggattacaggcgtaagccactgtgcctggtcttttttcttcttaagtacaggcatttgtacctatagatttccctgtaaacactgctttagctgcatcttgtaagttttggtttgttgtgtcttcattatcactcatctcaaagggttttgtaatttcccttatgatttttttctttgacacatttttttttttttttggtaatgacagggtcttgctgtgttgcccaggctggtcttgaattcctggtctcaagggatccaaggaatcctcccacttcggcctaccaaagtgctgagatttcaggcgtgagctactgcacccagccagtcacttacaagtgtgtctgatttccacatatttgtgagtttcccaacttttcattgttttctaacttcatcccatgtggtcagagggcatgctttgcatgatttcagtctacttatatttattaaggcttgttttatgctttaacttatgacctattttggagatgtttcatatgcactcgagaagaatatgtattctgatgttgggtggaaagttctatagatgtcttttaggtcaatttgccttataatgttgttcaagtcttctatttcctggtttatcttctgtctaggtgctctattattgaaaaaggggtattgaatattccaactctttttatggacttatctgtttctcctttcctttcagtttttgcttcatgtattttgggctctactgttagatgcatatatatttatagttgttacatcttcctgatgtattgacccttttatcattgtaacattttactctttatctccagtaacatttttttaagtctattttgtctggtattagaatagccactccagctttcttatggctgttgtctgtgtgatatatttgttttccatccttttacctttaatctctttctatcttctaaagtgtgtctcaaatagatggcatgaagtggaatcagacttgtttctgacatctctgccttttatagtattgcttaatccatgcacattgttattttgatataggaagacttatgactgccattttattgtttttgatatgcctcaagctttttgcttctccattccttcttttgcattatttcataatgtgatatttacatttaataatatttttgattttttaaaagttatttcctcagtggttgctctagggcttaccatacacatcttaactaaacagaataggcttcagataaacactaacttaattccaatgtaacaaccctattcctatataaacccatcccccgctttgtggtattattgttatatatgttattcctatacattacaaacccaacacacattattataattacttaatataattttacatctttaaaagaagctgagagaagagtaagtatatgtttatagtttttttatattaaacttatttcctatttcacgttctctccatttgttcctgtggatttgtcttaccatctggagtcagttctttagtacaagacagttttgcttccactcagcttcttcaacctgtagcacatgatatgagagaagtcgcttggagatttgaccgttgctttttgttctttccaaactctatcaccaatattttcccatgtagtttgtatccatttactagatgcaatgcttgccatgctatctccttattgggaaaggtgataaaagcctggcccctcattcgtccagtcatcattcggaattgaattggaggtccttttttctcctggaaccgagcgaacaatgacacaagatctctttcagtcacccgagggctaaggttcttcaggtataatacctctcataagttgaaactcttcaagacgttttttcattatcatctcttggtaaaaactttccaggttgttcatgggatcacctttgttcttcttttggggttcatcttttgtgcctaattttatcttcctcttcattgaggtcatgtacttgtctgcacttgtctttttgtggtatgcttggtaataaagagccttaaggaaggagtgacgatcagctccctgaaataaagacttttctatttccatttctcgccgggtcagctgtttgctctttgcaaatctctgtggcaggcaaagaatgcgctgacgctccgagatcctttcttcaatatcttgaagacggttctgtattgcttcaggagttgccctcagttttgtcttcttttcaccagaaacatggctcttccagatcaagatttctgtttcattaagccctaattccctgagagaagcagtttcctggtccttctcatgcagtgtctggaattgggacaaagtcatagtcccagctgcttccttcccaaagggcttgtacatagtaccaggagcaaagctctctttcttagacatacattcctcaatggagacagaagtatcaagttgatgctgaaggaggcttttcagctgcctctccccttctgtttccagctcctccaggacatgctcatcactcttcacacagctgtttaccatctccggcgccgggaatttgtcagcctcaaacccttttgcccagctgggtccgggtgaaacgacgaagccgcagcacccggccagctcccggggcccgtgccgggagggcattcccacagcagccggccccggtggcagcccttcctgaacttc

SEQ ID NO: 11254 - RNA, 2946 nt, Homo sapiens
  source 1..2946: mol_type = other RNA
ctgaatagctgggactacaggtgcccacgaccacgcctggctaattttttgtatttttagtagagacagggtttcaccatgttacccagaatggtctcgatctcctgaccccatgatctccacccgccccggcctcccaaagtgctgggattacaggcgtaagccactgtgcctggtcttttttcttcttaagtacaggcatttgtacctatagatttccctgtaaacactgctttagctgcatcttgtaagttttggtttgttgtgtcttcattatcactcatctcaaagggttttgtaatttcccttatgatttttttctttgacacatttttttttttttttggtaatgacagggtcttgctgtgttgcccaggctggtcttgaattcctggtctcaagggatccaaggaatcctcccacttcggcctaccaaagtgctgagatttcaggcgtgagctactgcacccagccagtcacttacaagtgtgtctgatttccacatatttgtgagtttcccaacttttcattgttttctaacttcatcccatgtggtcagagggcatgctttgcatgatttcagtctacttatatttattaaggcttgttttatgctttaacttatgacctattttggagatgtttcatatgcactcgagaagaatatgtattctgatgttgggtggaaagttctatagatgtcttttaggtcaatttgccttataatgttgttcaagtcttctatttcctggtttatcttctgtctaggtgctctattattgaaaaaggggtattgaatattccaactctttttatggacttatctgtttctcctttcctttcagtttttgcttcatgtattttgggctctactgttagatgcatatatatttatagttgttacatcttcctgatgtattgacccttttatcattgtaacattttactctttatctccagtaacatttttttaagtctattttgtctggtattagaatagccactccagctttcttatggctgttgtctgtgtgatatatttgttttccatccttttacctttaatctctttctatcttctaaagtgtgtctcaaatagatggcatgaagtggaatcagacttgtttctgacatctctgccttttatagtattgcttaatccatgcacattgttattttgatataggaagacttatgactgccattttattgtttttgatatgcctcaagctttttgcttctccattccttcttttgcattatttcataatgtgatatttacatttaataatatttttgattttttaaaagttatttcctcagtggttgctctagggcttaccatacacatcttaactaaacagaataggcttcagataaacactaacttaattccaatgtaacaaccctattcctatataaacccatcccccgctttgtggtattattgttatatatgttattcctatacattacaaacccaacacacattattataattacttaatataattttacatctttaaaagaagctgagagaagagtaagtatatgtttatagtttttttatattaaacttatttcctatttcacgttctctccatttgttcctgtggatttgtcttaccatctggagtcagttctttagtacaagacagttttgcttccactcagcttcttcaacctgtagcacatgatatgagagaagtcgcttggagatttgaccgttgctttttgttctttccaaactctatcaccaatattttcccatgtagtttgtatccatttactagatgcaatgcttgccatgctatctccttattgggaaaggtgataaaagcctggcccctcattcgtccagtcatcattcggaattgaattggaggtccttttttctcctggaaccgagcgaacaatgacacaagatctctttcagtcacccgagggctaaggttcttcaggtataataccttgtttggttcccctggattatatgaagaaaacataggaatttttcggatctcttcctctgacaaacgatttctctggatttcatcttctgggacaaattctattggctgcgtcagcttcttaggcccagtccaacactgctcaggtgaaaaatcaataacatttgccacatggagactggggcctttaccctgtgctgcctgttttcccttgtcctggagtaatgatgggctctcagctgtgccactatcacccactgatgtagctgagaccagtgagtgggaagcaaagggttcacctctcataagttgaaactcttcaagacgttttttcattatcatctcttggtaaaaactttccaggttgttcatgggatcacctttgttcttcttttggggttcatcttggtaataaagagccttaaggaaggagtgacgatcagctccctgaaataaagacttttctatttccatttctcgccgggtcagctgtttgctctttgcaaatctctgtggcaggcaaagaatgcgctgacgctccgagatcctttcttcaatatcttgaagacggttctgtattgcttcaggagttgccctcagttttgtcttcttttcaccagaaacatggctcttccagatcaagatttctgtttcattaagccctaattccctgagagaagcagtttcctggtccttctcatgcagtgtctggaattgggacaaagtcatagtcccagctgcttccttcccaaagggcttgtacatagtaccaggagcaaagctctctttcttagacatacattcctcaatggagacagaagtatcaagttgatgctgaaggaggcttttcagctgcctctccccttctgtttccagctcctccaggacatgctcatcactcttcacacagctgtttaccctcttcatgtttccacaggcccctacctccaacttgggtaaataggccgcggacctc

SEQ ID NO: 11255 - RNA, 3018 nt, Homo sapiens
  source 1..3018: mol_type = other RNA
ctgaatagctgggactacaggtgcccacgaccacgcctggctaattttttgtatttttagtagagacagggtttcaccatgttacccagaatggtctcgatctcctgaccccatgatctccacccgccccggcctcccaaagtgctgggattacaggcgtaagccactgtgcctggtcttttttcttcttaagtacaggcatttgtacctatagatttccctgtaaacactgctttagctgcatcttgtaagttttggtttgttgtgtcttcattatcactcatctcaaagggttttgtaatttcccttatgatttttttctttgacacatttttttttttttttggtaatgacagggtcttgctgtgttgcccaggctggtcttgaattcctggtctcaagggatccaaggaatcctcccacttcggcctaccaaagtgctgagatttcaggcgtgagctactgcacccagccagtcacttacaagtgtgtctgatttccacatatttgtgagtttcccaacttttcattgttttctaacttcatcccatgtggtcagagggcatgctttgcatgatttcagtctacttatatttattaaggcttgttttatgctttaacttatgacctattttggagatgtttcatatgcactcgagaagaatatgtattctgatgttgggtggaaagttctatagatgtcttttaggtcaatttgccttataatgttgttcaagtcttctatttcctggtttatcttctgtctaggtgctctattattgaaaaaggggtattgaatattccaactctttttatggacttatctgtttctcctttcctttcagtttttgcttcatgtattttgggctctactgttagatgcatatatatttatagttgttacatcttcctgatgtattgacccttttatcattgtaacattttactctttatctccagtaacatttttttaagtctattttgtctggtattagaatagccactccagctttcttatggctgttgtctgtgtgatatatttgttttccatccttttacctttaatctctttctatcttctaaagtgtgtctcaaatagatggcatgaagtggaatcagacttgtttctgacatctctgccttttatagtattgcttaatccatgcacattgttattttgatataggaagacttatgactgccattttattgtttttgatatgcctcaagctttttgcttctccattccttcttttgcattatttcataatgtgatatttacatttaataatatttttgattttttaaaagttatttcctcagtggttgctctagggcttaccatacacatcttaactaaacagaataggcttcagataaacactaacttaattccaatgtaacaaccctattcctatataaacccatcccccgctttgtggtattattgttatatatgttattcctatacattacaaacccaacacacattattataattacttaatataattttacatctttaaaagaagctgagagaagagtaagtatatgtttatagtttttttatattaaacttatttcctatttcacgttctctccatttgttcctgtggatttgtcttaccatctggagtcagttctttagtacaagacagttttgcttccactcagcttcttcaacctgtagcacatgatatgagagaagtcgcttggagatttgaccgttgctttttgttctttccaaactctatcaccaatattttcccatgtagtttgtatccatttactagatgcaatgcttgccatgctatctccttattgggaaaggtgataaaagcctggcccctcattcgtccagtcatcattcggaattgaattggaggtccttttttctcctggaaccgagcgaacaatgacacaagatctctttcagtcacccgagggctaaggttcttcaggtataataccttgtttggttcccctggattatatgaagaaaacataggaatttttcggatctcttcctctgacaaacgatttctctggatttcatcttctgggacaaattctattggctgcgtcagcttcttaggcccagtccaacactgctcaggtgaaaaatcaataacatttgccacatggagactggggcctttaccctgtgctgcctgttttcccttgtcctggagtaatgatgggctctcagctgtgccactatcacccactgatgtagctgagaccagtgagtgggaagcaaagggttcacctctcataagttgaaactcttcaagacgttttttcattatcatctcttggtaaaaactttccaggttgttcatgggatcacctttgttcttcttttggggttcatcttttgtgcctaattttatcttcctcttcattgaggtcatgtacttgtctgcacttgtctttttgtggtatgcttggtaataaagagccttaaggaaggagtgacgatcagctccctgaaataaagacttttctatttccatttctcgccgggtcagctgtttgctctttgcaaatctctgtggcaggcaaagaatgcgctgacgctccgagatcctttcttcaatatcttgaagacggttctgtattgcttcaggagttgccctcagttttgtcttcttttcaccagaaacatggctcttccagatcaagatttctgtttcattaagccctaattccctgagagaagcagtttcctggtccttctcatgcagtgtctggaattgggacaaagtcatagtcccagctgcttccttcccaaagggcttgtacatagtaccaggagcaaagctctctttcttagacatacattcctcaatggagacagaagtatcaagttgatgctgaaggaggcttttcagctgcctctccccttctgtttccagctcctccaggacatgctcatcactcttcacacagctgtttaccctcttcatgtttccacaggcccctacctccaacttgggtaaataggccgcggacctc

SEQ ID NO: 11256 - RNA, 5539 nt, Homo sapiens
  source 1..5539: mol_type = other RNA
ctgaatagctgggactacaggtgcccacgaccacgcctggctaattttttgtatttttagtagagacagggtttcaccatgttacccagaatggtctcgatctcctgaccccatgatctccacccgccccggcctcccaaagtgctgggattacaggcgtaagccactgtgcctggtcttttttcttcttaagtacaggcatttgtacctatagatttccctgtaaacactgctttagctgcatcttgtaagttttggtttgttgtgtcttcattatcactcatctcaaagggttttgtaatttcccttatgatttttttctttgacacatttttttttttttttggtaatgacagggtcttgctgtgttgcccaggctggtcttgaattcctggtctcaagggatccaaggaatcctcccacttcggcctaccaaagtgctgagatttcaggcgtgagctactgcacccagccagtcacttacaagtgtgtctgatttccacatatttgtgagtttcccaacttttcattgttttctaacttcatcccatgtggtcagagggcatgctttgcatgatttcagtctacttatatttattaaggcttgttttatgctttaacttatgacctattttggagatgtttcatatgcactcgagaagaatatgtattctgatgttgggtggaaagttctatagatgtcttttaggtcaatttgccttataatgttgttcaagtcttctatttcctggtttatcttctgtctaggtgctctattattgaaaaaggggtattgaatattccaactctttttatggacttatctgtttctcctttcctttcagtttttgcttcatgtattttgggctctactgttagatgcatatatatttatagttgttacatcttcctgatgtattgacccttttatcattgtaacattttactctttatctccagtaacatttttttaagtctattttgtctggtattagaatagccactccagctttcttatggctgttgtctgtgtgatatatttgttttccatccttttacctttaatctctttctatcttctaaagtgtgtctcaaatagatggcatgaagtggaatcagacttgtttctgacatctctgccttttatagtattgcttaatccatgcacattgttattttgatataggaagacttatgactgccattttattgtttttgatatgcctcaagctttttgcttctccattccttcttttgcattatttcataatgtgatatttacatttaataatatttttgattttttaaaagttatttcctcagtggttgctctagggcttaccatacacatcttaactaaacagaataggcttcagataaacactaacttaattccaatgtaacaaccctattcctatataaacccatcccccgctttgtggtattattgttatatatgttattcctatacattacaaacccaacacacattattataattacttaatataattttacatctttaaaagaagctgagagaagagtaagtatatgtttatagtttttttatattaaacttatttcctatttcacgttctctccatttgttcctgtggatttgtcttaccatctggagtcagttctttagtacaagacagttttgcttccactcagcttcttcaacctgttatcggcaaatatattatattttatacgttataggccaaacgatgcaactatatacatattgttttatacaactgtgttttacattagttaagagaaaaaagaaaaatgcatagattgtttctgataattacataattatttttgcctgtgctctttttctgcatgtgtgtagattcagattactgtctgtggtcacttgctttcaggctgaagaacttccttttgtatttccagcaagtcaggtctgccagcaacaaattctcttggtttttgattatgtgagatgttttatttcacgttcatttttgaaaaatagttttattgtatataggattattggttgacagttattttctttgaacactttgaatgtgttattccactgccactgccattgtttctgaggggaagtcaactactaattttatttgggttccttggtaagtgatggctcatttttctcgtattgctgttaagattttcttttcgtttttgggttttagcatttttcttatgatgtatctgtctgtaatttctttttcttctgggatgtataggttaatgtctctcatcaaatcgggggtatttatagccattatttcttagaatatttttctgctccttcatttcttttccttttttcctgtactcccattagaaatatgtaggaatgcttaatggtgtcacacaggttctatactcttgttcaattttattcattgttttcctttctgttcttcagcctggataatatctcagttcatcttcacaacccagtgaggtaagtagcattattatcctcactttatagatgaaaaatgtgaggctcagattaagtgacttgccaaggtcatagaatgttaagtgtggctgtacaggtctgactccagtttgtactacttcctctctgtatattgtttttttattttccagcaaccataaacaaacaactgggggatttgtgactggcatcctcttttctagagaacgctttatttccatttccgtttggcattctttgcttgtatgttcctcttctaaaattcatatgcctaatatttaacatatattagacacttaatcaatgtttattgctatgaattcaatgatactcaatggttgctagcttaaatggctgtgagaacaccaacattttgatctaaaatatttcactagaaaaatatatagctttttgaagactgataacttgtggaggaagcattcattaaataagtcaactgacttatgaaactacctactattactgctgatagttctgacttaatagcatttgttgatgcttaggcctgggggtcctactcttttatttactaggtggatgaaatatggcaaatgggctctagtaaagaaatatttcaacatttaattagttttttatttctgtgtatacgaagcagtctaagaaagaatgttatctctagagacaaatattgaggaccccagaaaaattataaagatttttaaaaatccttaggaataatccgttgtaattcatcctgagaaaataatactctttgcactttacccttcatactcagcatatcatctgtcctatatagtcttcaattatataatagaaaatgttttctaccagttctctccaaaagctgaaattacttttttcccctccctcagttagtttttcctcttcaactccaaacaaactggtgtctatacataaatcctagatccaagattccaattcaagaaagaccatccaggacccacaatttatatatattctagctaccactaatttctgtagtgctacctgtagcacatgatatgagagaagtcgcttggagatttgaccgttgctttttgttctttccaaactctatcaccaatattttcccatgtagtttgtatccatttactagatgcaatgcttgccatgctatctccttattgggaaaggtgataaaagcctggcccctcattcgtccagtcatcattcggaattgaattggaggtccttttttctcctggaaccgagcgaacaatgacacaagatctctttcagtcacccgagggctaaggttcttcaggtataatacctaaaacaaattgaggatcaaccaaaatatcatataaaggaggtaaggcactctttgtttttttctttttgagacaaagtctcactctgtcacccaggctggagtgcagtggcgcaatctctgctcactgcaaccttggcctcccaggctcaagtgattctcatgcctcagcctcccgagtagctgggattacagtcatgtgccaccacacctggctaatttttgtatttttagtagacgtggggtttcaccatgttgtccaggctggtcttgaactcccaaactcaggtgatccacccgccttggcctcccaaaatgctgggattacaggcgtgagacaccatgctcagccgtaagaaaactctttcattatgattagaattagtttcacataaaaatggtggattgaacacattcatttaatttcattccatccagaaaactctctaaaactataggcacttaaaaaaaaaaaaaaaaaaacacaaatcaacaaggtcaggaggaacaagaaaaggagacaacagcaataataatctggaagatgaaaaataattggatgagcaggaaccaactcagcacactgaagaaagctgaattttaaactggtagtggagagagccaagaacacacctgtcaccacttaagaatccttaaatagttcaggaactgataatttcacttaccttcagaaataaatgtgaagggatggggttaaaataaggcaaatcagttgaaggctgtctaaaagccaatatgatttttaaataccctccctcacaatatgctatggggtaaaagataacttgccaatcctggtagaaaacttgaggctcattgtcagaagatggggaatgccatacatggctgaagatgtgaacactgtttctgaaagcaaggaaactaagagaatactaaatgttgaggtcctcccagtccttttctgccatttggctcctagaacgctggtagtaccctcgtaagaaagattttggaagtcttctctgggaaaactggtaagtcctctcataagttgaaactcttcaagacgttttttcattatcatctcttggtaaaaactttccaggttgttcatgggatcacctttgttcttcttttggggttcatcttttgtgcctaattttatcttcctcttcattgaggtcatgtacttgtctgcacttgtctttttgtggtatgcttggtaataaagagccttaaggaaggagtgacgatcagctccctgaaataaagacttttctatttccatttctcgccgggtcagctgtttgctctttgcaaatctctgtggcaggcaaagaatgcgctgacgctccgagatcctttcttcaatatcttgaagacggttctgtattgcttcaggagttgccctcagttttgtcttcttttcaccagaaacatggctcttccagatcaagatttctgtttcattaagccctaattccctgagagaagcagtttcctggtccttctcatgcagtgtctggaattgggacaaagtcatagtcccagctgcttccttcccaaagggcttgtacatagtaccaggagcaaagctctctttcttagacatacattcctcaatggagacagaagtatcaagttgatgctgaaggaggcttttcagctgcctctccccttctgtttccagctcctccaggacatgctcatcactcttcacacagctgtttaccctcttcatgtttccacaggcccctacctccaacttgggtaaataggccgcggacctc

SEQ ID NO: 11257 - RNA, 4840 nt, Homo sapiens
  source 1..4840: mol_type = other RNA
ctgaatagctgggactacaggtgcccacgaccacgcctggctaattttttgtatttttagtagagacagggtttcaccatgttacccagaatggtctcgatctcctgaccccatgatctccacccgccccggcctcccaaagtgctgggattacaggcgtaagccactgtgcctggtcttttttcttcttaagtacaggcatttgtacctatagatttccctgtaaacactgctttagctgcatcttgtaagttttggtttgttgtgtcttcattatcactcatctcaaagggttttgtaatttcccttatgatttttttctttgacacatttttttttttttttggtaatgacagggtcttgctgtgttgcccaggctggtcttgaattcctggtctcaagggatccaaggaatcctcccacttcggcctaccaaagtgctgagatttcaggcgtgagctactgcacccagccagtcacttacaagtgtgtctgatttccacatatttgtgagtttcccaacttttcattgttttctaacttcatcccatgtggtcagagggcatgctttgcatgatttcagtctacttatatttattaaggcttgttttatgctttaacttatgacctattttggagatgtttcatatgcactcgagaagaatatgtattctgatgttgggtggaaagttctatagatgtcttttaggtcaatttgccttataatgttgttcaagtcttctatttcctggtttatcttctgtctaggtgctctattattgaaaaaggggtattgaatattccaactctttttatggacttatctgtttctcctttcctttcagtttttgcttcatgtattttgggctctactgttagatgcatatatatttatagttgttacatcttcctgatgtattgacccttttatcattgtaacattttactctttatctccagtaacatttttttaagtctattttgtctggtattagaatagccactccagctttcttatggctgttgtctgtgtgatatatttgttttccatccttttacctttaatctctttctatcttctaaagtgtgtctcaaatagatggcatgaagtggaatcagacttgtttctgacatctctgccttttatagtattgcttaatccatgcacattgttattttgatataggaagacttatgactgccattttattgtttttgatatgcctcaagctttttgcttctccattccttcttttgcattatttcataatgtgatatttacatttaataatatttttgattttttaaaagttatttcctcagtggttgctctagggcttaccatacacatcttaactaaacagaataggcttcagataaacactaacttaattccaatgtaacaaccctattcctatataaacccatcccccgctttgtggtattattgttatatatgttattcctatacattacaaacccaacacacattattataattacttaatataattttacatctttaaaagaagctgagagaagagtaagtatatgtttatagtttttttatattaaacttatttcctatttcacgttctctccatttgttcctgtggatttgtcttaccatctggagtcagttctttagtacaagacagttttgcttccactcagcttcttcaacctgttatcggcaaatatattatattttatacgttataggccaaacgatgcaactatatacatattgttttatacaactgtgttttacattagttaagagaaaaaagaaaaatgcatagattgtttctgataattacataattatttttgcctgtgctctttttctgcatgtgtgtagattcagattactgtctgtggtcacttgctttcaggctgaagaacttccttttgtatttccagcaagtcaggtctgccagcaacaaattctcttggtttttgattatgtgagatgttttatttcacgttcatttttgaaaaatagttttattgtatataggattattggttgacagttattttctttgaacactttgaatgtgttattccactgccactgccattgtttctgaggggaagtcaactactaattttatttgggttccttggtaagtgatggctcatttttctcgtattgctgttaagattttcttttcgtttttgggttttagcatttttcttatgatgtatctgtctgtaatttctttttcttctgggatgtataggttaatgtctctcatcaaatcgggggtatttatagccattatttcttagaatatttttctgctccttcatttcttttccttttttcctgtactcccattagaaatatgtaggaatgcttaatggtgtcacacaggttctatactcttgttcaattttattcattgttttcctttctgttcttcagcctggataatatctcagttcatcttcacaacccagtgaggtaagtagcattattatcctcactttatagatgaaaaatgtgaggctcagattaagtgacttgccaaggtcatagaatgttaagtgtggctgtacaggtctgactccagtttgtactacttcctctctgtatattgtttttttattttccagcaaccataaacaaacaactgggggatttgtgactggcatcctcttttctagagaacgctttatttccatttccgtttggcattctttgcttgtatgttcctcttctaaaattcatatgcctaatatttaacatatattagacacttaatcaatgtttattgctatgaattcaatgatactcaatggttgctagcttaaatggctgtgagaacaccaacattttgatctaaaatatttcactagaaaaatatatagctttttgaagactgataacttgtggaggaagcattcattaaataagtcaactgacttatgaaactacctactattactgctgatagttctgacttaatagcatttgttgatgcttaggcctgggggtcctactcttttatttactaggtggatgaaatatggcaaatgggctctagtaaagaaatatttcaacatttaattagttttttatttctgtgtatacgaagcagtctaagaaagaatgttatctctagagacaaatattgaggaccccagaaaaattataaagatttttaaaaatccttaggaataatccgttgtaattcatcctgagaaaataatactctttgcactttacccttcatactcagcatatcatctgtcctatatagtcttcaattatataatagaaaatgttttctaccagttctctccaaaagctgaaattacttttttcccctccctcagttagtttttcctcttcaactccaaacaaactggtgtctatacataaatcctagatccaagattccaattcaagaaagaccatccaggacccacaatttatatatattctagctaccactaatttctgtagtgctacctgtagcacatgatatgagagaagtcgcttggagatttgaccgttgctttttgttctttccaaactctatcaccaatattttcccatgtagtttgtatccatttactagatgcaatgcttgccatgctatctccttattgggaaaggtgataaaagcctggcccctcattcgtccagtcatcattcggaattgaattggaggtccttttttctcctggaaccgagcgaacaatgacacaagatctctttcagtcacccgagggctaaggttcttcaggtataataccttgtttggttcccctggattatatgaagaaaacataggaatttttcggatctcttcctctgacaaacgatttctctggatttcatcttctgggacaaattctattggctgcgtcagcttcttaggcccagtccaacactgctcaggtgaaaaatcaataacatttgccacatggagactggggcctttaccctgtgctgcctgttttcccttgtcctggagtaatgatgggctctcagctgtgccactatcacccactgatgtagctgagaccagtgagtgggaagcaaagggttcacctctcataagttgaaactcttcaagacgttttttcattatcatctcttggtaaaaactttccaggttgttcatgggatcacctttgttcttcttttggggttcatcttggtaataaagagccttaaggaaggagtgacgatcagctccctgaaataaagacttttctatttccatttctcgccgggtcagctgtttgctctttgcaaatctctgtggcaggcaaagaatgcgctgacgctccgagatcctttcttcaatatcttgaagacggttctgtattgcttcaggagttgccctcagttttgtcttcttttcaccagaaacatggctcttccagatcaagatttctgtttcattaagccctaattccctgagagaagcagtttcctggtccttctcatgcagtgtctggaattgggacaaagtcatagtcccagctgcttccttcccaaagggcttgtacatagtaccaggagcaaagctctctttcttagacatacattcctcaatggagacagaagtatcaagttgatgctgaaggaggcttttcagctgcctctccccttctgtttccagctcctccaggacatgctcatcactcttcacacagctgtttaccatctccggcgccgggaatttgtcagcctcaaacccttttgcccagctgggtccgggtgaaacgacgaagccgcagcacccggccagctcccggggcccgtgccgggagggcattcccacagcagccggccccggtggcagcccttcctgaactt

SEQ ID NO: 11258 - RNA, 4743 nt, Homo sapiens
  source 1..4743: mol_type = other RNA
ctgaatagctgggactacaggtgcccacgaccacgcctggctaattttttgtatttttagtagagacagggtttcaccatgttacccagaatggtctcgatctcctgaccccatgatctccacccgccccggcctcccaaagtgctgggattacaggcgtaagccactgtgcctggtcttttttcttcttaagtacaggcatttgtacctatagatttccctgtaaacactgctttagctgcatcttgtaagttttggtttgttgtgtcttcattatcactcatctcaaagggttttgtaatttcccttatgatttttttctttgacacatttttttttttttttggtaatgacagggtcttgctgtgttgcccaggctggtcttgaattcctggtctcaagggatccaaggaatcctcccacttcggcctaccaaagtgctgagatttcaggcgtgagctactgcacccagccagtcacttacaagtgtgtctgatttccacatatttgtgagtttcccaacttttcattgttttctaacttcatcccatgtggtcagagggcatgctttgcatgatttcagtctacttatatttattaaggcttgttttatgctttaacttatgacctattttggagatgtttcatatgcactcgagaagaatatgtattctgatgttgggtggaaagttctatagatgtcttttaggtcaatttgccttataatgttgttcaagtcttctatttcctggtttatcttctgtctaggtgctctattattgaaaaaggggtattgaatattccaactctttttatggacttatctgtttctcctttcctttcagtttttgcttcatgtattttgggctctactgttagatgcatatatatttatagttgttacatcttcctgatgtattgacccttttatcattgtaacattttactctttatctccagtaacatttttttaagtctattttgtctggtattagaatagccactccagctttcttatggctgttgtctgtgtgatatatttgttttccatccttttacctttaatctctttctatcttctaaagtgtgtctcaaatagatggcatgaagtggaatcagacttgtttctgacatctctgccttttatagtattgcttaatccatgcacattgttattttgatataggaagacttatgactgccattttattgtttttgatatgcctcaagctttttgcttctccattccttcttttgcattatttcataatgtgatatttacatttaataatatttttgattttttaaaagttatttcctcagtggttgctctagggcttaccatacacatcttaactaaacagaataggcttcagataaacactaacttaattccaatgtaacaaccctattcctatataaacccatcccccgctttgtggtattattgttatatatgttattcctatacattacaaacccaacacacattattataattacttaatataattttacatctttaaaagaagctgagagaagagtaagtatatgtttatagtttttttatattaaacttatttcctatttcacgttctctccatttgttcctgtggatttgtcttaccatctggagtcagttctttagtacaagacagttttgcttccactcagcttcttcaacctgttatcggcaaatatattatattttatacgttataggccaaacgatgcaactatatacatattgttttatacaactgtgttttacattagttaagagaaaaaagaaaaatgcatagattgtttctgataattacataattatttttgcctgtgctctttttctgcatgtgtgtagattcagattactgtctgtggtcacttgctttcaggctgaagaacttccttttgtatttccagcaagtcaggtctgccagcaacaaattctcttggtttttgattatgtgagatgttttatttcacgttcatttttgaaaaatagttttattgtatataggattattggttgacagttattttctttgaacactttgaatgtgttattccactgccactgccattgtttctgaggggaagtcaactactaattttatttgggttccttggtaagtgatggctcatttttctcgtattgctgttaagattttcttttcgtttttgggttttagcatttttcttatgatgtatctgtctgtaatttctttttcttctgggatgtataggttaatgtctctcatcaaatcgggggtatttatagccattatttcttagaatatttttctgctccttcatttcttttccttttttcctgtactcccattagaaatatgtaggaatgcttaatggtgtcacacaggttctatactcttgttcaattttattcattgttttcctttctgttcttcagcctggataatatctcagttcatcttcacaacccagtgaggtaagtagcattattatcctcactttatagatgaaaaatgtgaggctcagattaagtgacttgccaaggtcatagaatgttaagtgtggctgtacaggtctgactccagtttgtactacttcctctctgtatattgtttttttattttccagcaaccataaacaaacaactgggggatttgtgactggcatcctcttttctagagaacgctttatttccatttccgtttggcattctttgcttgtatgttcctcttctaaaattcatatgcctaatatttaacatatattagacacttaatcaatgtttattgctatgaattcaatgatactcaatggttgctagcttaaatggctgtgagaacaccaacattttgatctaaaatatttcactagaaaaatatatagctttttgaagactgataacttgtggaggaagcattcattaaataagtcaactgacttatgaaactacctactattactgctgatagttctgacttaatagcatttgttgatgcttaggcctgggggtcctactcttttatttactaggtggatgaaatatggcaaatgggctctagtaaagaaatatttcaacatttaattagttttttatttctgtgtatacgaagcagtctaagaaagaatgttatctctagagacaaatattgaggaccccagaaaaattataaagatttttaaaaatccttaggaataatccgttgtaattcatcctgagaaaataatactctttgcactttacccttcatactcagcatatcatctgtcctatatagtcttcaattatataatagaaaatgttttctaccagttctctccaaaagctgaaattacttttttcccctccctcagttagtttttcctcttcaactccaaacaaactggtgtctatacataaatcctagatccaagattccaattcaagaaagaccatccaggacccacaatttatatatattctagctaccactaatttctgtagtgctacctgtagcacatgatatgagagaagtcgcttggagatttgaccgttgctttttgttctttccaaactctatcaccaatattttcccatgtagtttgtatccatttactagatgcaatgcttgccatgctatctccttattgggaaaggtgataaaagcctggcccctcattcgtccagtcatcattcggaattgaattggaggtccttttttctcctggaaccgagcgaacaatgacacaagatctctttcagtcacccgagggctaaggttcttcaggtataataccttgtttggttcccctggattatatgaagaaaacataggaatttttcggatctcttcctctgacaaacgatttctctggatttcatcttctgggacaaattctattggctgcgtcagcttcttaggcccagtccaacactgctcaggtgaaaaatcaataacatttgccacatggagactggggcctttaccctgtgctgcctgttttcccttgtcctggagtaatgatgggctctcagctgtgccactatcacccactgatgtagctgagaccagtgagtgggaagcaaagggttcacctctcataagttgaaactcttcaagacgttttttcattatcatctcttggtaaaaactttccaggttgttcatgggatcacctttgttcttcttttggggttcatcttggtaataaagagccttaaggaaggagtgacgatcagctccctgaaataaagacttttctatttccatttctcgccgggtcagctgtttgctctttgcaaatctctgtggcaggcaaagaatgcgctgacgctccgagatcctttcttcaatatcttgaagacggttctgtattgcttcaggagttgccctcagttttgtcttcttttcaccagaaacatggctcttccagatcaagatttctgtttcattaagccctaattccctgagagaagcagtttcctggtccttctcatgcagtgtctggaattgggacaaagtcatagtcccagctgcttccttcccaaagggcttgtacatagtaccaggagcaaagctctctttcttagacatacattcctcaatggagacagaagtatcaagttgatgctgaaggaggcttttcagctgcctctccccttctgtttccagctcctccaggacatgctcatcactcttcacacagctgtttaccctcttcatgtttccacaggcccctacctccaacttgggtaaataggccgcggacctc

SEQ ID NO: 11259 - RNA, 4913 nt, Homo sapiens
  source 1..4913: mol_type = other RNA
ctgaatagctgggactacaggtgcccacgaccacgcctggctaattttttgtatttttagtagagacagggtttcaccatgttacccagaatggtctcgatctcctgaccccatgatctccacccgccccggcctcccaaagtgctgggattacaggcgtaagccactgtgcctggtcttttttcttcttaagtacaggcatttgtacctatagatttccctgtaaacactgctttagctgcatcttgtaagttttggtttgttgtgtcttcattatcactcatctcaaagggttttgtaatttcccttatgatttttttctttgacacatttttttttttttttggtaatgacagggtcttgctgtgttgcccaggctggtcttgaattcctggtctcaagggatccaaggaatcctcccacttcggcctaccaaagtgctgagatttcaggcgtgagctactgcacccagccagtcacttacaagtgtgtctgatttccacatatttgtgagtttcccaacttttcattgttttctaacttcatcccatgtggtcagagggcatgctttgcatgatttcagtctacttatatttattaaggcttgttttatgctttaacttatgacctattttggagatgtttcatatgcactcgagaagaatatgtattctgatgttgggtggaaagttctatagatgtcttttaggtcaatttgccttataatgttgttcaagtcttctatttcctggtttatcttctgtctaggtgctctattattgaaaaaggggtattgaatattccaactctttttatggacttatctgtttctcctttcctttcagtttttgcttcatgtattttgggctctactgttagatgcatatatatttatagttgttacatcttcctgatgtattgacccttttatcattgtaacattttactctttatctccagtaacatttttttaagtctattttgtctggtattagaatagccactccagctttcttatggctgttgtctgtgtgatatatttgttttccatccttttacctttaatctctttctatcttctaaagtgtgtctcaaatagatggcatgaagtggaatcagacttgtttctgacatctctgccttttatagtattgcttaatccatgcacattgttattttgatataggaagacttatgactgccattttattgtttttgatatgcctcaagctttttgcttctccattccttcttttgcattatttcataatgtgatatttacatttaataatatttttgattttttaaaagttatttcctcagtggttgctctagggcttaccatacacatcttaactaaacagaataggcttcagataaacactaacttaattccaatgtaacaaccctattcctatataaacccatcccccgctttgtggtattattgttatatatgttattcctatacattacaaacccaacacacattattataattacttaatataattttacatctttaaaagaagctgagagaagagtaagtatatgtttatagtttttttatattaaacttatttcctatttcacgttctctccatttgttcctgtggatttgtcttaccatctggagtcagttctttagtacaagacagttttgcttccactcagcttcttcaacctgttatcggcaaatatattatattttatacgttataggccaaacgatgcaactatatacatattgttttatacaactgtgttttacattagttaagagaaaaaagaaaaatgcatagattgtttctgataattacataattatttttgcctgtgctctttttctgcatgtgtgtagattcagattactgtctgtggtcacttgctttcaggctgaagaacttccttttgtatttccagcaagtcaggtctgccagcaacaaattctcttggtttttgattatgtgagatgttttatttcacgttcatttttgaaaaatagttttattgtatataggattattggttgacagttattttctttgaacactttgaatgtgttattccactgccactgccattgtttctgaggggaagtcaactactaattttatttgggttccttggtaagtgatggctcatttttctcgtattgctgttaagattttcttttcgtttttgggttttagcatttttcttatgatgtatctgtctgtaatttctttttcttctgggatgtataggttaatgtctctcatcaaatcgggggtatttatagccattatttcttagaatatttttctgctccttcatttcttttccttttttcctgtactcccattagaaatatgtaggaatgcttaatggtgtcacacaggttctatactcttgttcaattttattcattgttttcctttctgttcttcagcctggataatatctcagttcatcttcacaacccagtgaggtaagtagcattattatcctcactttatagatgaaaaatgtgaggctcagattaagtgacttgccaaggtcatagaatgttaagtgtggctgtacaggtctgactccagtttgtactacttcctctctgtatattgtttttttattttccagcaaccataaacaaacaactgggggatttgtgactggcatcctcttttctagagaacgctttatttccatttccgtttggcattctttgcttgtatgttcctcttctaaaattcatatgcctaatatttaacatatattagacacttaatcaatgtttattgctatgaattcaatgatactcaatggttgctagcttaaatggctgtgagaacaccaacattttgatctaaaatatttcactagaaaaatatatagctttttgaagactgataacttgtggaggaagcattcattaaataagtcaactgacttatgaaactacctactattactgctgatagttctgacttaatagcatttgttgatgcttaggcctgggggtcctactcttttatttactaggtggatgaaatatggcaaatgggctctagtaaagaaatatttcaacatttaattagttttttatttctgtgtatacgaagcagtctaagaaagaatgttatctctagagacaaatattgaggaccccagaaaaattataaagatttttaaaaatccttaggaataatccgttgtaattcatcctgagaaaataatactctttgcactttacccttcatactcagcatatcatctgtcctatatagtcttcaattatataatagaaaatgttttctaccagttctctccaaaagctgaaattacttttttcccctccctcagttagtttttcctcttcaactccaaacaaactggtgtctatacataaatcctagatccaagattccaattcaagaaagaccatccaggacccacaatttatatatattctagctaccactaatttctgtagtgctacctgtagcacatgatatgagagaagtcgcttggagatttgaccgttgctttttgttctttccaaactctatcaccaatattttcccatgtagtttgtatccatttactagatgcaatgcttgccatgctatctccttattgggaaaggtgataaaagcctggcccctcattcgtccagtcatcattcggaattgaattggaggtccttttttctcctggaaccgagcgaacaatgacacaagatctctttcagtcacccgagggctaaggttcttcaggtataataccttgtttggttcccctggattatatgaagaaaacataggaatttttcggatctcttcctctgacaaacgatttctctggatttcatcttctgggacaaattctattggctgcgtcagcttcttaggcccagtccaacactgctcaggtgaaaaatcaataacatttgccacatggagactggggcctttaccctgtgctgcctgttttcccttgtcctggagtaatgatgggctctcagctgtgccactatcacccactgatgtagctgagaccagtgagtgggaagcaaagggttcacctctcataagttgaaactcttcaagacgttttttcattatcatctcttggtaaaaactttccaggttgttcatgggatcacctttgttcttcttttggggttcatcttttgtgcctaattttatcttcctcttcattgaggtcatgtacttgtctgcacttgtctttttgtggtatgcttggtaataaagagccttaaggaaggagtgacgatcagctccctgaaataaagacttttctatttccatttctcgccgggtcagctgtttgctctttgcaaatctctgtggcaggcaaagaatgcgctgacgctccgagatcctttcttcaatatcttgaagacggttctgtattgcttcaggagttgccctcagttttgtcttcttttcaccagaaacatggctcttccagatcaagatttctgtttcattaagccctaattccctgagagaagcagtttcctggtccttctcatgcagtgtctggaattgggacaaagtcatagtcccagctgcttccttcccaaagggcttgtacatagtaccaggagcaaagctctctttcttagacatacattcctcaatggagacagaagtatcaagttgatgctgaaggaggcttttcagctgcctctccccttctgtttccagctcctccaggacatgctcatcactcttcacacagctgtttaccatctccggcgccgggaatttgtcagcctcaaacccttttgcccagctgggtccgggtgaaacgacgaagccgcagcacccggccagctcccggggcccgtgccgggagggcattcccacagcagccggccccggtggcagcccttcctgaacttc

SEQ ID NO: 11260 - RNA, 4815 nt, Homo sapiens
  source 1..4815: mol_type = other RNA
ctgaatagctgggactacaggtgcccacgaccacgcctggctaattttttgtatttttagtagagacagggtttcaccatgttacccagaatggtctcgatctcctgaccccatgatctccacccgccccggcctcccaaagtgctgggattacaggcgtaagccactgtgcctggtcttttttcttcttaagtacaggcatttgtacctatagatttccctgtaaacactgctttagctgcatcttgtaagttttggtttgttgtgtcttcattatcactcatctcaaagggttttgtaatttcccttatgatttttttctttgacacatttttttttttttttggtaatgacagggtcttgctgtgttgcccaggctggtcttgaattcctggtctcaagggatccaaggaatcctcccacttcggcctaccaaagtgctgagatttcaggcgtgagctactgcacccagccagtcacttacaagtgtgtctgatttccacatatttgtgagtttcccaacttttcattgttttctaacttcatcccatgtggtcagagggcatgctttgcatgatttcagtctacttatatttattaaggcttgttttatgctttaacttatgacctattttggagatgtttcatatgcactcgagaagaatatgtattctgatgttgggtggaaagttctatagatgtcttttaggtcaatttgccttataatgttgttcaagtcttctatttcctggtttatcttctgtctaggtgctctattattgaaaaaggggtattgaatattccaactctttttatggacttatctgtttctcctttcctttcagtttttgcttcatgtattttgggctctactgttagatgcatatatatttatagttgttacatcttcctgatgtattgacccttttatcattgtaacattttactctttatctccagtaacatttttttaagtctattttgtctggtattagaatagccactccagctttcttatggctgttgtctgtgtgatatatttgttttccatccttttacctttaatctctttctatcttctaaagtgtgtctcaaatagatggcatgaagtggaatcagacttgtttctgacatctctgccttttatagtattgcttaatccatgcacattgttattttgatataggaagacttatgactgccattttattgtttttgatatgcctcaagctttttgcttctccattccttcttttgcattatttcataatgtgatatttacatttaataatatttttgattttttaaaagttatttcctcagtggttgctctagggcttaccatacacatcttaactaaacagaataggcttcagataaacactaacttaattccaatgtaacaaccctattcctatataaacccatcccccgctttgtggtattattgttatatatgttattcctatacattacaaacccaacacacattattataattacttaatataattttacatctttaaaagaagctgagagaagagtaagtatatgtttatagtttttttatattaaacttatttcctatttcacgttctctccatttgttcctgtggatttgtcttaccatctggagtcagttctttagtacaagacagttttgcttccactcagcttcttcaacctgttatcggcaaatatattatattttatacgttataggccaaacgatgcaactatatacatattgttttatacaactgtgttttacattagttaagagaaaaaagaaaaatgcatagattgtttctgataattacataattatttttgcctgtgctctttttctgcatgtgtgtagattcagattactgtctgtggtcacttgctttcaggctgaagaacttccttttgtatttccagcaagtcaggtctgccagcaacaaattctcttggtttttgattatgtgagatgttttatttcacgttcatttttgaaaaatagttttattgtatataggattattggttgacagttattttctttgaacactttgaatgtgttattccactgccactgccattgtttctgaggggaagtcaactactaattttatttgggttccttggtaagtgatggctcatttttctcgtattgctgttaagattttcttttcgtttttgggttttagcatttttcttatgatgtatctgtctgtaatttctttttcttctgggatgtataggttaatgtctctcatcaaatcgggggtatttatagccattatttcttagaatatttttctgctccttcatttcttttccttttttcctgtactcccattagaaatatgtaggaatgcttaatggtgtcacacaggttctatactcttgttcaattttattcattgttttcctttctgttcttcagcctggataatatctcagttcatcttcacaacccagtgaggtaagtagcattattatcctcactttatagatgaaaaatgtgaggctcagattaagtgacttgccaaggtcatagaatgttaagtgtggctgtacaggtctgactccagtttgtactacttcctctctgtatattgtttttttattttccagcaaccataaacaaacaactgggggatttgtgactggcatcctcttttctagagaacgctttatttccatttccgtttggcattctttgcttgtatgttcctcttctaaaattcatatgcctaatatttaacatatattagacacttaatcaatgtttattgctatgaattcaatgatactcaatggttgctagcttaaatggctgtgagaacaccaacattttgatctaaaatatttcactagaaaaatatatagctttttgaagactgataacttgtggaggaagcattcattaaataagtcaactgacttatgaaactacctactattactgctgatagttctgacttaatagcatttgttgatgcttaggcctgggggtcctactcttttatttactaggtggatgaaatatggcaaatgggctctagtaaagaaatatttcaacatttaattagttttttatttctgtgtatacgaagcagtctaagaaagaatgttatctctagagacaaatattgaggaccccagaaaaattataaagatttttaaaaatccttaggaataatccgttgtaattcatcctgagaaaataatactctttgcactttacccttcatactcagcatatcatctgtcctatatagtcttcaattatataatagaaaatgttttctaccagttctctccaaaagctgaaattacttttttcccctccctcagttagtttttcctcttcaactccaaacaaactggtgtctatacataaatcctagatccaagattccaattcaagaaagaccatccaggacccacaatttatatatattctagctaccactaatttctgtagtgctacctgtagcacatgatatgagagaagtcgcttggagatttgaccgttgctttttgttctttccaaactctatcaccaatattttcccatgtagtttgtatccatttactagatgcaatgcttgccatgctatctccttattgggaaaggtgataaaagcctggcccctcattcgtccagtcatcattcggaattgaattggaggtccttttttctcctggaaccgagcgaacaatgacacaagatctctttcagtcacccgagggctaaggttcttcaggtataataccttgtttggttcccctggattatatgaagaaaacataggaatttttcggatctcttcctctgacaaacgatttctctggatttcatcttctgggacaaattctattggctgcgtcagcttcttaggcccagtccaacactgctcaggtgaaaaatcaataacatttgccacatggagactggggcctttaccctgtgctgcctgttttcccttgtcctggagtaatgatgggctctcagctgtgccactatcacccactgatgtagctgagaccagtgagtgggaagcaaagggttcacctctcataagttgaaactcttcaagacgttttttcattatcatctcttggtaaaaactttccaggttgttcatgggatcacctttgttcttcttttggggttcatcttttgtgcctaattttatcttcctcttcattgaggtcatgtacttgtctgcacttgtctttttgtggtatgcttggtaataaagagccttaaggaaggagtgacgatcagctccctgaaataaagacttttctatttccatttctcgccgggtcagctgtttgctctttgcaaatctctgtggcaggcaaagaatgcgctgacgctccgagatcctttcttcaatatcttgaagacggttctgtattgcttcaggagttgccctcagttttgtcttcttttcaccagaaacatggctcttccagatcaagatttctgtttcattaagccctaattccctgagagaagcagtttcctggtccttctcatgcagtgtctggaattgggacaaagtcatagtcccagctgcttccttcccaaagggcttgtacatagtaccaggagcaaagctctctttcttagacatacattcctcaatggagacagaagtatcaagttgatgctgaaggaggcttttcagctgcctctccccttctgtttccagctcctccaggacatgctcatcactcttcacacagctgtttaccctcttcatgtttccacaggcccctacctccaacttgggtaaataggccgcggacctc

SEQ ID NO: 11261 - RNA, 4505 nt, Homo sapiens
  source 1..4505: mol_type = other RNA
ctgaatagctgggactacaggtgcccacgaccacgcctggctaattttttgtatttttagtagagacagggtttcaccatgttacccagaatggtctcgatctcctgaccccatgatctccacccgccccggcctcccaaagtgctgggattacaggcgtaagccactgtgcctggtcttttttcttcttaagtacaggcatttgtacctatagatttccctgtaaacactgctttagctgcatcttgtaagttttggtttgttgtgtcttcattatcactcatctcaaagggttttgtaatttcccttatgatttttttctttgacacatttttttttttttttggtaatgacagggtcttgctgtgttgcccaggctggtcttgaattcctggtctcaagggatccaaggaatcctcccacttcggcctaccaaagtgctgagatttcaggcgtgagctactgcacccagccagtcacttacaagtgtgtctgatttccacatatttgtgagtttcccaacttttcattgttttctaacttcatcccatgtggtcagagggcatgctttgcatgatttcagtctacttatatttattaaggcttgttttatgctttaacttatgacctattttggagatgtttcatatgcactcgagaagaatatgtattctgatgttgggtggaaagttctatagatgtcttttaggtcaatttgccttataatgttgttcaagtcttctatttcctggtttatcttctgtctaggtgctctattattgaaaaaggggtattgaatattccaactctttttatggacttatctgtttctcctttcctttcagtttttgcttcatgtattttgggctctactgttagatgcatatatatttatagttgttacatcttcctgatgtattgacccttttatcattgtaacattttactctttatctccagtaacatttttttaagtctattttgtctggtattagaatagccactccagctttcttatggctgttgtctgtgtgatatatttgttttccatccttttacctttaatctctttctatcttctaaagtgtgtctcaaatagatggcatgaagtggaatcagacttgtttctgacatctctgccttttatagtattgcttaatccatgcacattgttattttgatataggaagacttatgactgccattttattgtttttgatatgcctcaagctttttgcttctccattccttcttttgcattatttcataatgtgatatttacatttaataatatttttgattttttaaaagttatttcctcagtggttgctctagggcttaccatacacatcttaactaaacagaataggcttcagataaacactaacttaattccaatgtaacaaccctattcctatataaacccatcccccgctttgtggtattattgttatatatgttattcctatacattacaaacccaacacacattattataattacttaatataattttacatctttaaaagaagctgagagaagagtaagtatatgtttatagtttttttatattaaacttatttcctatttcacgttctctccatttgttcctgtggatttgtcttaccatctggagtcagttctttagtacaagacagttttgcttccactcagcttcttcaacctgttatcggcaaatatattatattttatacgttataggccaaacgatgcaactatatacatattgttttatacaactgtgttttacattagttaagagaaaaaagaaaaatgcatagattgtttctgataattacataattatttttgcctgtgctctttttctgcatgtgtgtagattcagattactgtctgtggtcacttgctttcaggctgaagaacttccttttgtatttccagcaagtcaggtctgccagcaacaaattctcttggtttttgattatgtgagatgttttatttcacgttcatttttgaaaaatagttttattgtatataggattattggttgacagttattttctttgaacactttgaatgtgttattccactgccactgccattgtttctgaggggaagtcaactactaattttatttgggttccttggtaagtgatggctcatttttctcgtattgctgttaagattttcttttcgtttttgggttttagcatttttcttatgatgtatctgtctgtaatttctttttcttctgggatgtataggttaatgtctctcatcaaatcgggggtatttatagccattatttcttagaatatttttctgctccttcatttcttttccttttttcctgtactcccattagaaatatgtaggaatgcttaatggtgtcacacaggttctatactcttgttcaattttattcattgttttcctttctgttcttcagcctggataatatctcagttcatcttcacaacccagtgaggtaagtagcattattatcctcactttatagatgaaaaatgtgaggctcagattaagtgacttgccaaggtcatagaatgttaagtgtggctgtacaggtctgactccagtttgtactacttcctctctgtatattgtttttttattttccagcaaccataaacaaacaactgggggatttgtgactggcatcctcttttctagagaacgctttatttccatttccgtttggcattctttgcttgtatgttcctcttctaaaattcatatgcctaatatttaacatatattagacacttaatcaatgtttattgctatgaattcaatgatactcaatggttgctagcttaaatggctgtgagaacaccaacattttgatctaaaatatttcactagaaaaatatatagctttttgaagactgataacttgtggaggaagcattcattaaataagtcaactgacttatgaaactacctactattactgctgatagttctgacttaatagcatttgttgatgcttaggcctgggggtcctactcttttatttactaggtggatgaaatatggcaaatgggctctagtaaagaaatatttcaacatttaattagttttttatttctgtgtatacgaagcagtctaagaaagaatgttatctctagagacaaatattgaggaccccagaaaaattataaagatttttaaaaatccttaggaataatccgttgtaattcatcctgagaaaataatactctttgcactttacccttcatactcagcatatcatctgtcctatatagtcttcaattatataatagaaaatgttttctaccagttctctccaaaagctgaaattacttttttcccctccctcagttagtttttcctcttcaactccaaacaaactggtgtctatacataaatcctagatccaagattccaattcaagaaagaccatccaggacccacaatttatatatattctagctaccactaatttctgtagtgctacctgtagcacatgatatgagagaagtcgcttggagatttgaccgttgctttttgttctttccaaactctatcaccaatattttcccatgtagtttgtatccatttactagatgcaatgcttgccatgctatctccttattgggaaaggtgataaaagcctggcccctcattcgtccagtcatcattcggaattgaattggaggtccttttttctcctggaaccgagcgaacaatgacacaagatctctttcagtcacccgagggctaaggttcttcaggtataataccttttgtgcctaattttatcttcctcttcattgaggtcatgtacttgtctgcacttgtctttttgtggtatgcttggtaataaagagccttaaggaaggagtgacgatcagctccctgaaataaagacttttctatttccatttctcgccgggtcagctgtttgctctttgcaaatctctgtggcaggcaaagaatgcgctgacgctccgagatcctttcttcaatatcttgaagacggttctgtattgcttcaggagttgccctcagttttgtcttcttttcaccagaaacatggctcttccagatcaagatttctgtttcattaagccctaattccctgagagaagcagtttcctggtccttctcatgcagtgtctggaattgggacaaagtcatagtcccagctgcttccttcccaaagggcttgtacatagtaccaggagcaaagctctctttcttagacatacatcagcaaattttctcttacatcttatttctaagctgaagcaccactgcaacaaaatggaactccatcgagagtgccgtcatccaggaataataaatcctcaatggagacagaagtatcaagttgatgctgaaggaggcttttcagctgcctctccccttctgtttccagctcctccaggacatgctcatcactcttcacacagctgtttaccctcttcatgtttccacaggcccctacctccaacttgggtaaataggccgcggacctc

SEQ ID NO: 11262 - RNA, 4509 nt, Homo sapiens
  source 1..4509: mol_type = other RNA
ctgaatagctgggactacaggtgcccacgaccacgcctggctaattttttgtatttttagtagagacagggtttcaccatgttacccagaatggtctcgatctcctgaccccatgatctccacccgccccggcctcccaaagtgctgggattacaggcgtaagccactgtgcctggtcttttttcttcttaagtacaggcatttgtacctatagatttccctgtaaacactgctttagctgcatcttgtaagttttggtttgttgtgtcttcattatcactcatctcaaagggttttgtaatttcccttatgatttttttctttgacacatttttttttttttttggtaatgacagggtcttgctgtgttgcccaggctggtcttgaattcctggtctcaagggatccaaggaatcctcccacttcggcctaccaaagtgctgagatttcaggcgtgagctactgcacccagccagtcacttacaagtgtgtctgatttccacatatttgtgagtttcccaacttttcattgttttctaacttcatcccatgtggtcagagggcatgctttgcatgatttcagtctacttatatttattaaggcttgttttatgctttaacttatgacctattttggagatgtttcatatgcactcgagaagaatatgtattctgatgttgggtggaaagttctatagatgtcttttaggtcaatttgccttataatgttgttcaagtcttctatttcctggtttatcttctgtctaggtgctctattattgaaaaaggggtattgaatattccaactctttttatggacttatctgtttctcctttcctttcagtttttgcttcatgtattttgggctctactgttagatgcatatatatttatagttgttacatcttcctgatgtattgacccttttatcattgtaacattttactctttatctccagtaacatttttttaagtctattttgtctggtattagaatagccactccagctttcttatggctgttgtctgtgtgatatatttgttttccatccttttacctttaatctctttctatcttctaaagtgtgtctcaaatagatggcatgaagtggaatcagacttgtttctgacatctctgccttttatagtattgcttaatccatgcacattgttattttgatataggaagacttatgactgccattttattgtttttgatatgcctcaagctttttgcttctccattccttcttttgcattatttcataatgtgatatttacatttaataatatttttgattttttaaaagttatttcctcagtggttgctctagggcttaccatacacatcttaactaaacagaataggcttcagataaacactaacttaattccaatgtaacaaccctattcctatataaacccatcccccgctttgtggtattattgttatatatgttattcctatacattacaaacccaacacacattattataattacttaatataattttacatctttaaaagaagctgagagaagagtaagtatatgtttatagtttttttatattaaacttatttcctatttcacgttctctccatttgttcctgtggatttgtcttaccatctggagtcagttctttagtacaagacagttttgcttccactcagcttcttcaacctgttatcggcaaatatattatattttatacgttataggccaaacgatgcaactatatacatattgttttatacaactgtgttttacattagttaagagaaaaaagaaaaatgcatagattgtttctgataattacataattatttttgcctgtgctctttttctgcatgtgtgtagattcagattactgtctgtggtcacttgctttcaggctgaagaacttccttttgtatttccagcaagtcaggtctgccagcaacaaattctcttggtttttgattatgtgagatgttttatttcacgttcatttttgaaaaatagttttattgtatataggattattggttgacagttattttctttgaacactttgaatgtgttattccactgccactgccattgtttctgaggggaagtcaactactaattttatttgggttccttggtaagtgatggctcatttttctcgtattgctgttaagattttcttttcgtttttgggttttagcatttttcttatgatgtatctgtctgtaatttctttttcttctgggatgtataggttaatgtctctcatcaaatcgggggtatttatagccattatttcttagaatatttttctgctccttcatttcttttccttttttcctgtactcccattagaaatatgtaggaatgcttaatggtgtcacacaggttctatactcttgttcaattttattcattgttttcctttctgttcttcagcctggataatatctcagttcatcttcacaacccagtgaggtaagtagcattattatcctcactttatagatgaaaaatgtgaggctcagattaagtgacttgccaaggtcatagaatgttaagtgtggctgtacaggtctgactccagtttgtactacttcctctctgtatattgtttttttattttccagcaaccataaacaaacaactgggggatttgtgactggcatcctcttttctagagaacgctttatttccatttccgtttggcattctttgcttgtatgttcctcttctaaaattcatatgcctaatatttaacatatattagacacttaatcaatgtttattgctatgaattcaatgatactcaatggttgctagcttaaatggctgtgagaacaccaacattttgatctaaaatatttcactagaaaaatatatagctttttgaagactgataacttgtggaggaagcattcattaaataagtcaactgacttatgaaactacctactattactgctgatagttctgacttaatagcatttgttgatgcttaggcctgggggtcctactcttttatttactaggtggatgaaatatggcaaatgggctctagtaaagaaatatttcaacatttaattagttttttatttctgtgtatacgaagcagtctaagaaagaatgttatctctagagacaaatattgaggaccccagaaaaattataaagatttttaaaaatccttaggaataatccgttgtaattcatcctgagaaaataatactctttgcactttacccttcatactcagcatatcatctgtcctatatagtcttcaattatataatagaaaatgttttctaccagttctctccaaaagctgaaattacttttttcccctccctcagttagtttttcctcttcaactccaaacaaactggtgtctatacataaatcctagatccaagattccaattcaagaaagaccatccaggacccacaatttatatatattctagctaccactaatttctgtagtgctacctgtagcacatgatatgagagaagtcgcttggagatttgaccgttgctttttgttctttccaaactctatcaccaatattttcccatgtagtttgtatccatttactagatgcaatgcttgccatgctatctccttattgggaaaggtgataaaagcctggcccctcattcgtccagtcatcattcggaattgaattggaggtccttttttctcctggaaccgagcgaacaatgacacaagatctctttcagtcacccgagggctaaggttcttcaggtataataccttttgtgcctaattttatcttcctcttcattgaggtcatgtacttgtctgcacttgtctttttgtggtatgcttggtaataaagagccttaaggaaggagtgacgatcagctccctgaaataaagacttttctatttccatttctcgccgggtcagctgtttgctctttgcaaatctctgtggcaggcaaagaatgcgctgacgctccgagatcctttcttcaatatcttgaagacggttctgtattgcttcaggagttgccctcagttttgtcttcttttcaccagaaacatggctcttccagatcaagatttctgtttcattaagccctaattccctgagagaagcagtttcctggtccttctcatgcagtgtctggaattgggacaaagtcatagtcccagctgcttccttcccaaagggcttgtacatagtaccaggagcaaagctctctttcttagacatacattcctcaatggagacagaagtatcaagttgatgctgaaggaggcttttcagctgcctctccccttctgtttccagctcctccaggacatgctcatcactcttcacacagctgtttaccatctccggcgccgggaatttgtcagcctcaaacccttttgcccagctgggtccgggtgaaacgacgaagccgcagcacccggccagctcccggggcccgtgccgggagggcattcccacagcagccggccccggtggcagcccttcctgaacttc

SEQ ID NO: 11263 - RNA, 4411 nt, Homo sapiens
  source 1..4411: mol_type = other RNA
ctgaatagctgggactacaggtgcccacgaccacgcctggctaattttttgtatttttagtagagacagggtttcaccatgttacccagaatggtctcgatctcctgaccccatgatctccacccgccccggcctcccaaagtgctgggattacaggcgtaagccactgtgcctggtcttttttcttcttaagtacaggcatttgtacctatagatttccctgtaaacactgctttagctgcatcttgtaagttttggtttgttgtgtcttcattatcactcatctcaaagggttttgtaatttcccttatgatttttttctttgacacatttttttttttttttggtaatgacagggtcttgctgtgttgcccaggctggtcttgaattcctggtctcaagggatccaaggaatcctcccacttcggcctaccaaagtgctgagatttcaggcgtgagctactgcacccagccagtcacttacaagtgtgtctgatttccacatatttgtgagtttcccaacttttcattgttttctaacttcatcccatgtggtcagagggcatgctttgcatgatttcagtctacttatatttattaaggcttgttttatgctttaacttatgacctattttggagatgtttcatatgcactcgagaagaatatgtattctgatgttgggtggaaagttctatagatgtcttttaggtcaatttgccttataatgttgttcaagtcttctatttcctggtttatcttctgtctaggtgctctattattgaaaaaggggtattgaatattccaactctttttatggacttatctgtttctcctttcctttcagtttttgcttcatgtattttgggctctactgttagatgcatatatatttatagttgttacatcttcctgatgtattgacccttttatcattgtaacattttactctttatctccagtaacatttttttaagtctattttgtctggtattagaatagccactccagctttcttatggctgttgtctgtgtgatatatttgttttccatccttttacctttaatctctttctatcttctaaagtgtgtctcaaatagatggcatgaagtggaatcagacttgtttctgacatctctgccttttatagtattgcttaatccatgcacattgttattttgatataggaagacttatgactgccattttattgtttttgatatgcctcaagctttttgcttctccattccttcttttgcattatttcataatgtgatatttacatttaataatatttttgattttttaaaagttatttcctcagtggttgctctagggcttaccatacacatcttaactaaacagaataggcttcagataaacactaacttaattccaatgtaacaaccctattcctatataaacccatcccccgctttgtggtattattgttatatatgttattcctatacattacaaacccaacacacattattataattacttaatataattttacatctttaaaagaagctgagagaagagtaagtatatgtttatagtttttttatattaaacttatttcctatttcacgttctctccatttgttcctgtggatttgtcttaccatctggagtcagttctttagtacaagacagttttgcttccactcagcttcttcaacctgttatcggcaaatatattatattttatacgttataggccaaacgatgcaactatatacatattgttttatacaactgtgttttacattagttaagagaaaaaagaaaaatgcatagattgtttctgataattacataattatttttgcctgtgctctttttctgcatgtgtgtagattcagattactgtctgtggtcacttgctttcaggctgaagaacttccttttgtatttccagcaagtcaggtctgccagcaacaaattctcttggtttttgattatgtgagatgttttatttcacgttcatttttgaaaaatagttttattgtatataggattattggttgacagttattttctttgaacactttgaatgtgttattccactgccactgccattgtttctgaggggaagtcaactactaattttatttgggttccttggtaagtgatggctcatttttctcgtattgctgttaagattttcttttcgtttttgggttttagcatttttcttatgatgtatctgtctgtaatttctttttcttctgggatgtataggttaatgtctctcatcaaatcgggggtatttatagccattatttcttagaatatttttctgctccttcatttcttttccttttttcctgtactcccattagaaatatgtaggaatgcttaatggtgtcacacaggttctatactcttgttcaattttattcattgttttcctttctgttcttcagcctggataatatctcagttcatcttcacaacccagtgaggtaagtagcattattatcctcactttatagatgaaaaatgtgaggctcagattaagtgacttgccaaggtcatagaatgttaagtgtggctgtacaggtctgactccagtttgtactacttcctctctgtatattgtttttttattttccagcaaccataaacaaacaactgggggatttgtgactggcatcctcttttctagagaacgctttatttccatttccgtttggcattctttgcttgtatgttcctcttctaaaattcatatgcctaatatttaacatatattagacacttaatcaatgtttattgctatgaattcaatgatactcaatggttgctagcttaaatggctgtgagaacaccaacattttgatctaaaatatttcactagaaaaatatatagctttttgaagactgataacttgtggaggaagcattcattaaataagtcaactgacttatgaaactacctactattactgctgatagttctgacttaatagcatttgttgatgcttaggcctgggggtcctactcttttatttactaggtggatgaaatatggcaaatgggctctagtaaagaaatatttcaacatttaattagttttttatttctgtgtatacgaagcagtctaagaaagaatgttatctctagagacaaatattgaggaccccagaaaaattataaagatttttaaaaatccttaggaataatccgttgtaattcatcctgagaaaataatactctttgcactttacccttcatactcagcatatcatctgtcctatatagtcttcaattatataatagaaaatgttttctaccagttctctccaaaagctgaaattacttttttcccctccctcagttagtttttcctcttcaactccaaacaaactggtgtctatacataaatcctagatccaagattccaattcaagaaagaccatccaggacccacaatttatatatattctagctaccactaatttctgtagtgctacctgtagcacatgatatgagagaagtcgcttggagatttgaccgttgctttttgttctttccaaactctatcaccaatattttcccatgtagtttgtatccatttactagatgcaatgcttgccatgctatctccttattgggaaaggtgataaaagcctggcccctcattcgtccagtcatcattcggaattgaattggaggtccttttttctcctggaaccgagcgaacaatgacacaagatctctttcagtcacccgagggctaaggttcttcaggtataataccttttgtgcctaattttatcttcctcttcattgaggtcatgtacttgtctgcacttgtctttttgtggtatgcttggtaataaagagccttaaggaaggagtgacgatcagctccctgaaataaagacttttctatttccatttctcgccgggtcagctgtttgctctttgcaaatctctgtggcaggcaaagaatgcgctgacgctccgagatcctttcttcaatatcttgaagacggttctgtattgcttcaggagttgccctcagttttgtcttcttttcaccagaaacatggctcttccagatcaagatttctgtttcattaagccctaattccctgagagaagcagtttcctggtccttctcatgcagtgtctggaattgggacaaagtcatagtcccagctgcttccttcccaaagggcttgtacatagtaccaggagcaaagctctctttcttagacatacattcctcaatggagacagaagtatcaagttgatgctgaaggaggcttttcagctgcctctccccttctgtttccagctcctccaggacatgctcatcactcttcacacagctgtttaccctcttcatgtttccacaggcccctacctccaacttgggtaaataggccgcggacctc

SEQ ID NO: 11264 - RNA, 1934 nt, Homo sapiens
  source 1..1934: mol_type = other RNA
ctgaatagctgggactacaggtgcccacgaccacgcctggctaatttttttgtattttttttagtagagacggggtttcaccgtgttcgccaggatggtctcgatctcctgaccttgtgatccgcccaccttggcctcccaaagtgctgggattacaggcgtgagccaccgcgcccagcctgccatgggcttttttaagacggagtttcactcttgtcgcccaggctggagtgcagtggcgcgatcttagctcacgcaacctccacctcctgggttcaagtgattctcttgcttcagcctcccaccaccatgccaggctaatttttgtatttttagtagagatggggtttcgccatgttggtcaggctggtctcgaactcctgacctcaggtgatccacctgcctcggcctcccaaagtactggcattaacaggcgtaagccactgtgcccggacaagcatgggccttttcttacaacaccaacaggaagaagtccttggaaagtttacttggagcaactctaaggtcctccaccttcaggaaatttagccaagctcaagtcaacagtttccttcccttctatctacaatagggaggtacttatgacagggacaaggacaatgaatcagaagtagcacccacccaggcaggttcccttcctcaagtttttagctccctggtcttagccagcaggcgacgatcccctcaagtttgccttttcctgtgacattgacagacctcaggacggactatagatcttctctgaccatggaaagacccagaagccatctcagaagattgggccctgctattcctccctgtcaggaacagtcatttcattaccaaccttggaccagagtctgtttgatgatctgaggaagtgtatgcatttttctttaaagctattttgatttagattaatgagatttttgcaaatgccttggcatataataggcaaactggcagctaggattcacagtctgcagaggtgaacaaaagggcccacacacctctgcatgatactactacatcccagggcatgtcctcctctgtagctcagtgaccctggtttccgcccacctccaaatcctgactagataagctcagctctggagcctgcttctccctcagtgcagtaaggatgtggctcgccagcgcaacgtccgaggaggtctctctgctgatacccgtgtctactgcatccacctcctcaccaaaggcagctttggactcttcctgctttgacaagaggctgccctctttctccaaagcctggaggtacagctgcaggagctgcttggactgacgcacttcctctctttggtcaagcacctgttggagtgtgtgctgcagccgctggacggtggcacaactctgacgtagttcctgagccaggtctgagcagggagcgtcaacaagcatctggaggtcctcctctgataggaggatgatgctggacagatcttctttcagctgcctggccacattcttccacttcaaccctgccccgctgtctgtttcatctacatcaaaggactcttgggaaatccaagctgtacctccatctgaattgttgtatgcccatttctcattactagccaatgccacaaacttagtattggaaggtagacacagaaagtaatcgtcatcatccactatggtgccatcctctgccaggaccagggtgactggtgtcagggacttatcaatggccagaatgtcacaggccttgctcctcaggtcttcgaggcaggaggcggccacgccgtgctgttcgcggctgtagttgcggcgcagcagacacggctttagagtccggatctcgccagattctggtaccccggcgtccccggtcacctccatcctccacaaggtgggacctgcccaccttcgagaagtcgcgggaggccggagcggcggtccttctactcgac

SEQ ID NO: 11265 - RNA, 4318 nt, Homo sapiens
  source 1..4318: mol_type = other RNA
ctgaatagctgggactacaggtgcccactaccacacctggctaatttttgtagagacgggttttcaccatgttgccaaggctggtctaaaactcctgagcccaagtgattcacctgccttggcctcccaaagtgctgggattacaggtgtgaaccactgcagccggcctcgaatctcataaatagtaatcatttctaaggtcaatggtattttctggttattcaaaactaaagagtttaagacaatatatggtactctcattcatgtatgctaactgactttagagttgtaagatgtgcacagtgtggataaagtagcagaaagattcccaatgtgggaaaaagggaaagtgttttatgggcttttagtacattgatatacccttcttgacagcaacatcagaatggagcaaaaaacataaggatgttcaacttttaactgagtgatctcactcttgagaaaaatgtaatagatgagaagctgaatgcatgagggtattcccagcagtgctctataatataacaaataatgaaaaactacctcagtggacaagaagagaagtagtgattaatgtgataacagcatctgaaacaaaatctatgatacaataactttaacaaataaaaacaagactagatagcaacatggaaaagcttgtgatataatgttcatggcttaaacaatgtaatgataacaatataaagtatatattcatgtaaacaaaaaccagtcatacaaaaatgaaaacagttattgttgttaacattgattattaatttttaaccttattgagatgttatctttttaattaaacagcaataggagttatttattaatcataccaatttcttttctaagttccagtagatagtgctactaaatccatttggaacactaaaaagaagacttgtgggttttatccgagttaggtatcctgataaatcattaccactttggtgattcacagaatacttcaaggtaccttccaaggaggtctggtggagccacggttaaccttttttccttgctgagccggtgcccttggatgaattcactcatggaaggggggcccttcagaagaaatgattctgtggaggtgggatcagggggaactcttaataaattctgtaggtaggaagcccctgaagtcctgggacggctctgatcacaaagggaaggtgaaaattgtcttttcctctgagtgccactgctgacccgaatgttgggtgtctgtgggccctgactatgcaggaggtaagtgtctatggtgggcacggtgactgatgcctccccacttactttagggctgccgatcttgctctttccaagtttgcctttgctgcgtcgggactgctcatggtcaaactctaagtcctccagcctctgggtcagggcgagtttttgctggatagccattcgtaacaaagtgttcagagtcttcttctcatcctctgcagctgctaactgtctctgcatctcatccaactgggtgacatattcatcacatcttgttgcaaacattgctctcagggatgagaaggttgcagcatcttctttcaaagccttcagttcatttctaagcttcgtcatggtttcagtcaccattgctttttcattttcatatttgttcttgagattagctagcgccacctcagctgtctgcttgttggctttcaacaccgccctcaatgtggcgatctgctcccgtttggtgctcagcagggactttagcttgaggatctcttccattaaggcttccttgtctttatcaatcatgggggctagctcccgagccgctgctctttgacgagacagttgcaaggaccggtccacagctttctgcagatgcttgatttggtcccggattatggcattaaggttgtagatattcattggctctttgcggatgtcacttgtatccaatactggagatgacggtggggcagtaataacaggagagattgtgggggtcttagttggacttggttctttgctggcctctgtgctttcttttgcaactggttcagatgaggtccttgtttctaccggggatgacacaccccgcctggctaatcgtggggacaaaagtcctctgggatcatcgggccctttcaggctgccactgcgggtgactctgctctgcctatagtaatccagcatgaccctgttgggagtttcattattacatagacacacatggtggtaaagctgagctaactcctcactgaatgtcactaactcatcctgggccgtattaagggtactgtgattttcgttggctatgctggtcatcttttgcaactccttctccatgtgggccatcttctcaccactctccttggtggtcttctcaaggcttgtcacctgctcatcatacatctggattttactctcatacttggccttctcatcagtgtagttttctacagatttattatatttctcctttaaggccttaatttcagctttcagatcaatcacctcagttactgccaccctgtatttgcattcaaggatctctaaaccattgatgtccacctcatagtcatgggcctcctcccctgagtcccggcccttctccccgtccagctcagccttgagctccttgctgctttgcaggcccctcatggcattgacgtgctctgtgagccggtgcacccgctcatgctgctccgtcagtgcccccttggtgtgttccagctgtgtctgtgactcctgtaggttggccaaaagaatggccttttcccgctctacctgcataagctgctgcttcaacttctgtatttctgaaatgttcagctcactgaataagtcagagacagggttcagagactctcctttccttaaggtgggagtccgatagtctccattcagtttcacaagaggcccatggatatgaccgttcattttgtcatcattgtttggttcactcccatcctcggcaaatttgagtccatctactgagatgctgatatggttatcattgaggctgatatactgggagagctccttccgcaggttgttcttttgctctctttcattttttaaagtctcgagggcttcttccagttggtgctcagcaatctctttcaatcggatggcatcttccagctggctgttcagcagtaccgtctcctcctcaaatcgcttaatctcatgctttaagccttcgtattcaacctggttctgcttcaacgtggacactagtttctgcaatgtgatattttcttcttccaattcagtatagtcctgaaggagccgtgcctcccggaacttatattctcggatttcatccttcatccgtattctctgtagctccaccatctcattgttctccttcagatcctgcacgactgcggtgagcctctcgttttctgcctgtacattagtgaccacagcccggctctgtttcagctcgttctgcatctccaagatcttccccagatagtaagcctccttcgatgctgactcctgcagaagcgtttcctcccgagtctctccatcttcagcaaccttccggtggatggagaaggactgcccaaatgcctctttgagctgctccagctcctgtttgaggctgtcgtactcagcctccagttcatcatactgctgtttgagggtcagcttctcctccagcaccaccagcccgtactcggcagcctggatcttctcgtgggtggtctccgtgagctccttggttagcctctctatctcagtcttataatggtccaccgtctgcaatacctcttctgcggccatagccccggtggatggaggcaggagggggttacggggtgggggagatggatgcgaagctggcggggaaagggagaaggaaatgggaagggatgggtggaaacggaaaagaaagtgcggccggatgaatgagcagcgcgatgccccgccggctctggtggcagcggcagctacaccgcccgagaaactgacgagaaatgcaacatggagaacagggcagagggtcaggggcgaggcggcaaaggccgccgcatgtgtcctcggggccggcccctgcgtgcggtcagcagccgtgcggcatggcccgggctgcggcggccgcgggtagcgaggggctccggattctgcttattcagagacgcccgtccgccatgtctcccgggccgcgtcactgcagtctcgccctgggtctggcgcgctccggctcgcggctcgctctctcgctccacctgctccctctggccctgcagcagccggtgcggaatgatgcagtctcggggccggctccctcccttcccgcgtggcggcggctccgagcagggggcggggagcggatggagtc

SEQ ID NO: 11266 - RNA, 4252 nt, Homo sapiens
  source 1..4252: mol_type = other RNA
ctgaatagctgggactacaggtgcccactgccgtgcccggctaattttttgtatttttagtagagacagggtttcaccgtgttagccaggatgctctcgatctcttgacctcaggtgatccacctgcctcggcctcccaaagtgctgggattacaggcgtgagccaccgcgcccagcctaactttaaaatgggggacaaaaaactgaacatactgacatattgattctttgaagagaaatctagaactcactgtaaccaacagaagaacttaaggcctggtgaatgaagtatctgaacctccaggtagatttttagtaagcacggagcctatgatgggtactggtttaaagccctaagggtggtcttagtttagttgaagaaaaggaaagaagatgtccttgaatcattattcagggtcaaggaatgagaggtgttggtgaaacaggcagagaggggacgtgatattagattaatgtcacatcattgcatcctatggaaggacctgtaatgttgttaggcagttgctaagggcaaattacaggaaaaatattaactggttaatagaatcatgtagtgataatagagagctgaaggcactttcagagatgatccggcccagctctctctctgcaggcaagggaatgtctaaatcatccaggacagatattgttgacatctcaaaaagctcattaagcataaagagtcctccacattttggggtagcccatctgattattttatcatcagaaggttaaaaaaatctcatccttacccaatctaaaactcagattggttaggtttttattttcttttacacaaccagccacaaactggtgcttatgatgatggtgtcttgtaaatgaacaacaaagagcagggaccactcgaccttcttactgcatgccttctttgtctcagagaaccagtgaggttcatttgctccacaaaaatttatcaagtaccaagctctgtgataggagctaaggatgaaggaatgaataaagtggaatccctgccctcaatccatttgagtctagtgggatgggagcagacaagtagagaggtaatatttaccaggtaatgtgttaactgtagtaacgttttttataaacatgagagtatttatcaaatgctgggaattgaggactaagctctgatttttttcttatcttagccaaattcctatctaaaggggtctggagagtcatgccctacaaaccataaattctcatcagatgggttttatttaagcctatatatcgtgatttactttccaatctgactcttgcataacattatgtgacaaacaagaaaataaaaatattttatcccaaaacatgtttctttgctgtattttgaaatggccgtgcaaagctgtcctttgtggcagaaaatttgcatctgtaaagaaactctattaacatagctagatctttttcttccaggccctcccagtcctgaagaggttaacggagagtctagcaccttttaaaggtctgaataggaaacgtttgtcttctgttgtctctaagggcagccactatgagacttcaaaagaaccttggtctccagaatcttaacctgaacatgaaattgacctatagcctggaagcctgccccaccccacgagttgtcccgctgttctggaccaagccaatatatttcttaatgtatctgattgatgtctcatgacttcctgaccaccttgggtacatgttctcaggatctcctgatggatgtgccagaggccatggtcactcatatttggctcagaataaatcttttcaaatattttacagcttgactcttttcagcgacaataattgtgctaagtgcttcaggcatattatcccattcattctcacaactcccttgtcactgtcgggccgttgagcccaacctaagccatcatatcccctgtgacctgcatgtatgcatccagatggcctgaagcaagtgaagaatcacaaaagaagtgaaaatggccagttcttgcattaactgatgacatttcaccattgtgatttgttcctgccccaccttaactgagcgattaaccttgtgaaattccttttcctgactcagaacctcccccactgagcaccttgtgacccccgcccctgcccgcaagagaacaaccccctttgactgtaattttccactactcacccaaatcctataaaagtgccccacccctatctccctttgctgactctcttttcggactcagcctgcctgcacctaggtgaaataaacagccttgttgctcacacaaagcctgtttggtggtctcttcacacagacgtgcgtgacagtcacaaacttatgattgcaaaaaaaccctttgagtgcaaccttttctttctggttggaacttattgttttgtagttttggtttttttgtttgtttgttttggtctgtttattttttatttatattggcttttttgttgcctttttcagttttatttctgtggttgaaactttatggcacattctaaattcttcctggcaatggcttagtgtgaatttatgatcagtcctgctagttttgcttgttagatgtaaaggaaatttttgaggctttagaaatcccttttctctctcaaatttataggctttcaagactgttgtttctatgggtttcaaaatcctatgctggcagtcaaaaactttctttctctttgcatttctgcagtaattctaattctcccggaggcaggtggaatcctctggaatgtcatatgcaagcaagtgaggaagaaaaaagaaagaggacatgttttaacatatcatctctcttttacaaaataaatggacacacacagacacttacacagttattgactcgaggagtcgctgcacattctcatataaaggtattacatcttaactagagatagttcttaaacttgcaaaatatagattacttctaatcacgtcatgtcaggcatcaatgtactgggtaagggtttcttttcccccctgtaattttttctactttgttgaacacattgagctaaaaaatcctatacgaagttgttcctttaggtaaattagttaattttcaataaaattacagctttcgtaaaatattaacaggcacttttgtctcttctgcatttctgcattggactccccgcatatctataccacacatatgtatgattattgttctctaaagcagtaattatgctgatagtaatgatcccgaatgaccgtaaagattgtctctgattacatttaacagcaaatacaaagacactgtttttcctacttgggtatatttaacagcaaatggtatgaacgatccagacagctgtaatggctgagttgggaagtctgtttcctgaatagggtagaaattcaccactggggaaagaaatgcttccccgttacttttattgtgttactgacccatcacatatgctcaggcttccaagctgagaacgtgccaaactattaaccaaaataatacgtctggctcccaaagctcacattttgtgtaaatgcaaatgtaatcccgaggtgtattagttagcaagatggccgtctggtgggacacttggtatcatgtgcccttcccgctccatggcttggaatggaatttgtgctggccgttaacgttcttgaatgcatttccctctgagcttggatagagggtaagacagccaaatggaaacatcttctttcaggttctttggaaatacatttattgatctctctcaatctttggcgggattttctttcttcctggatgaacaggaacaactctgggagccgcttgcagtgacacgatgcagctgtgtgtatacctggatgccatatgggaaactgcaaattcagcaaaagggaaggcaatgctgaaattcaccttcaaagctaaatattgttccttagaccaatttcaacctcgaattcatttgaatttcctttatgtctggttacatctatttttttttctagattctgtgctcattagctctcttacagctttcactcaaacatgcacttagcccctagaacctcaagataatccctgttctccaagtatgcttctgcatgactgtccttgaaaatccacagatgactgtccatgaaaatccacagatctcctgttcctttgggtcttcattttctgaaagttcccgtgtcacataataccttccatccatatctggatctaacatttccttcaacaggtggtgataaagaggccacgaggcactcagagaagcacagcaagtaagt

SEQ ID NO: 11267 - RNA, 3110 nt, Homo sapiens
  source 1..3110: mol_type = other RNA
ctgaatagctgggactacaggtgcccatcaccacacctggctaatttttttctatttttagtagagatgggttttcaccatgttagccaggatggtctcgatctcctgacctcgtgatccagccacctcggcctcccaaagtgctgggattacaggcgtaagccaccatgcctggccgatcactttaactcctactgggccatgtgaaattctgaagtttgaacattagaaacaccagtttagaagaagtttaacaaggaagtgggcaggggaccacctctccaaggtataaggtcagaggtacccagaaatgcctctcctattcgtgccccatcaaaggacagttcttggggggttgtgagacaatgtgtgaattcccatggtaccattcttgtgggcctaagcatttgagactgtcaacaaaatgggaagagcttcagggaagagtgacaggcaaggctgcgatcaaacattcactcaaggggatgggacactgaaccgtcacacctccatgagccagaaggccagtgagagcctaagctacctgctgggcggtgtccacggaggggggaaaagatacaatgtataaagatacaatgtaactgatgatacaatgtaactctcaccacgaatttggataaggcaactagtcagaaccacttagcaagatagcttctttggcaaaaaggaatcaagagtttggtagacatggttcaagggtagcgatttgggtcagggctccccaaacttgagcatgcatgtgcacgaatcacctagggcagtgcatgaaagttggattctaatcagtgggcctggggtgaggcctgggagtctgcatttctaaccagcgccccagaaatgccaggcctgccggcccaaggaccacacttggggtatcgagggtctccaaagtctgcatctgattacctattttactaacagtaaaactgatacttatctccaagattaaatacttcatgtacatcaatgcagaatgtctcctttgtctccagtctaatggtttctaaatcttccgttctcgttccatcaagttctgtaacgaatacaccctcagtggccacagcctggggagtcggttcttccctggcagctcccaggggcggtggtggtggggcctcagctgggagggtcccctctggctctcgatctccatcctctcctttaaccttcacaggcggtgacagtagcagggtctcagctgggagggtcccctctggctcttgatctccatcctctcctttaacctccacaggtggcgggggtggtggggcctcagctgggagggtcccctctggctctccatctccgtcctctcctttaacctccacaggtgacgacagtagcagggtctcagctgggagggtcccctctggctctggacctccatcctctcttttagcctccacaggcggctcctctccacttggcttttccgggcagagctcgtccttggcctcaaagctttccttaacaaatagctccatcttctgccttgtttctctgtccccgggaggctcctccttgccttccgcactggcgggcacattctcaccatcatctgaagatgtcatctcccctctctcttgactctctctctgtcttttcctctcctctgcccgctgcttgatcatggccaaggcttcaatgctgtctgtgatcttcttccgctccctgctctcccactgctgtctctcctccttttcagctgcgtaccctcccctagcccaggcctccgcacaagctctgtcctttggaaacactggtctatcatccaggtatgttaagtgctttagtcgtacagtgactgtccttctgtaattaggaatctgtctgataaccgggtttcccatcaaattcagtacacgcaaatcgggcatgctttccagaatgctcaggatctccgggtcactcagcttgttgtgcgaaaggtcaaggacacaaagcctcaaacactcttgtagatgctgaatgtcctccacggtctccaggtgattgtgggccatctgcaatgtgttcaggactgggaggcaggagaggttttcaatggtcttgatgtaattgttgctgaggttaagagcatccagtttctgcagaggttccaggttctcaattttacggagcaagttcatttgcaagaagaggcaacgcaactcagtttgggcctccaggttttcgattttctgtattccattgctctgcagccagagacagcgcagccctgtgtactcttccaggttctcaatgcgatcaaaacctttaaagtgtaaatacagcgtatcattcaatgctggggtaatataaagcttgtgctgcttgcagagtttttgcagggaacttttagtcattctggggccccgatcttccctgtcttctcttgggtgtgcgaagtgaccacctgacccattatcaccactctgtttctgctggctgtggtaggatgtgtcagaagaacccacacatatttccttaggatcattaatttctgatgatccgcccgcctcggcctcccaaagtgctggaattacaggcgttgagccaccgcacccggccaagtctcttctgtcactgactagccgagggttatctgtttggtgcaagttttgtaacctcttaagtatgtttcctcctcagtacgaaatggcgagagaagcccctactgcagagcgttgcttgctaccattattattattgttattatttggctgtgaagatcgggtatgtggtgtgggaagggggctggagcgcctagccgtgtctgcccctcgcccaccgccctccctggggggcagtcggcaccttccttgcagccccctcggcctgcgctcccgtggtcacccgcagactcctccacgccgggctcctgcgcgcaatccagctctgctgcaccacctgtcgcaggctccgagggctcagggtgcatgtttacttcggcgacaccgaacgccccgcagctttggggggcccaggttcgcggcggacgtcgctacggccccagcccagccagagagtaccctctttccttcttcgccagccgctggcgccctagtctttacagcccaacgcttccccggtcgcccaggcaaccgctg

SEQ ID NO: 11268 - RNA, 5890 nt, Homo sapiens
  source 1..5890: mol_type = other RNA
ctgaatagctgggactacaggtgcccgacaacatgcctggctaattttttgtattgttagtaaagacggggtttcaccgtgttagccaggctgttctcgatctcctgacctcgtgatccacccgcctcggcctcccaaagtgtagggattacaggcgtgagccaccacacccagcccagaatgctttttctataaaaggtatccatgtatttcaccagtcagagatgtactaggtaaggaaaaaacaaaacaaataaacaaaaaaaatcacctcaagttttggaggcaggattgacctgggtttgaatcccagatctgactctttgtcatgtgataagctagagtctccaaggctcaatttcatcttcaaaatggggatagacaccaccttccttgggtttaaaggattaagaaagatgatatatgagatggtgctcaaaaagatcagtctattcctttcaacatgcctgtaaatgtatttctagggcatgtaaaagccaagtcgctcacattcagaaagagtaggcacttctaaaacaagtcccgggccaggtgtgcacagccatctgcacaggctgtgaacagaggcgtgcacagctcctgggggtagccctcatgctcccgcaggatcctctttaacaaagctgattcataaaagctgtcacccattacgcctgtgttctataattttgtgagccttttcacatgaaagactacccaagggtaggccgggtacggtggctcacgcctataatcccagcagtttggcaggccgaggcaggcggatcacctgaagtcgggagtttgagaccagcctgaccaaaatggagaaacctcgtctctaccaaaaatacaaaatcagccggacgtggtagcgcatgcctgtattcccaactactcaggaaggctaatgcaggagaatcgcttgaacccgggaggcggaggttgcggtgagctgagatcgcgccattgtactccagcctgggcaacaagagcaaaactccgtctcaaaaaaaaaaaaaagactactcaaggtagaaggaatccccattgcaaaaataaaaataaaaaaaaagtgctcaaatcatcagagtcagggagacatacaccagaacagaattccaggctgcgggctcacagcctccacactgctgacagttggggcagaccattctttgctcaggggacagtcctgtgcattatggcatgtttaacagtatcttactagatgccagtggcatcccactctcagtcgtgccaaccaaaatgcctccacacacagccaagtgtccccagcagacacaagccccctgagttaagagccctggttaagagtggaatggtgtaagggaatgtttgtgctcctccaacagccagtcccaaacatgcgctaatgtcatttcatccttaaccttgtgtggttgctgtcatctccacattacagatgggggaaatgaggcccagagttctgacgcaatcatccaaggtctcttagaaaatacgttgtagaaccagcatccaaaccagttctgttgggctaagtggggcccctccgctatgcaatactatccttttaaaataagagctcattcccagacacagaatctttctagaatcttactgggttactagccaaccaatatttactaataaggtatacatacatgatctatggcctaatttgaaattgaagatgattaccaaaaataattatgctgggcttacagtaaataatcttatgctattagtttctggcaaaaccagacatacaactggcctgctgagctgacccgttctctgtcgatgaccataggctatgtcatgggtataatggagcggcccacacacatggcctcaggacagctgctgcctccacacctgcaccccctgggtcccactgtgctagcagtttacacacgtcagctcctgtgatccttaaaacaacgctctgaggtaggagtaatcacccccatttcacagaggaggaaagtgagactcagagaaagtaggtaacttgctggtaagtggctgagccatgatcaaagtgttttggtcaccaaagttcttacatgtgaacccctgcactgtacagcattgtacatgacggggcaggttatagagaggggaggctaggtccagtgcggtagctcacgcctgtaatcccagcactttgggaggctgaggcaggtggatcactgtcaggcctctgagcccaagctaagccatcatatccccagtgacctgcatgtatacatccagatggcctgaagcaactgaagatccacaaaagaagtgaaaatagccttaactgatgacattccaccattgtgatttgtttctgccccaccctaactatcaatgtactttgtaatctcccccacacttaagaaggttctttataatctcccccacccttaagaaggtttttttgtaattctccccacccttgagaatgtactttgtgagatccaccccctgcccccaaaacattgctcttaactccactgcctatcccaaaacctgtaagaactaatgataatcccaccaccctttgctgactctcttttcagactcagcctgcctgcacccaggtgaaataaacagccttgttacttacacaaagcctgtttggtctcttcacacggacatgtaagacaatcacgaggtcaggagttcaagaccagcctggccaaaattgtgaaaccccatctctacaaaaaatacaaaaattagcctggcatggtggcatgcgcctgtaatcccagctactctagaggttgaagcaggagaattgcttaaacctgggggggcagaggctgtagtgagccgagatcgcgccactgcactccagcctgggcgacagagcaagactccatctcgaaaaaaaaaaaagagagaggggaccatgtcctggcttcattctgctggaaacagtcatgccaggcaggcccaaatggttgaacttctttttcctctcacagtaaaatccaaagcggggcaggtcccatggtacgctcccccaggaggatcatgggttcctccttgggactgtaggacgaaggaagcagctagcaaaggcgttcgctcaaagctactgtgtgcaataggtatgctggagggtcaggctggagcgtggggtggggtaagaccctctgaaagtttactctctgtcactgttgcctctcaagaggttctgatgctacgagaaagtgaaggtgatcaggaaggacaagctgtaggtgaagtatcattttcaaaaagtcatttaaaactgcaaactgccaaatgcggcagctcatgcctgtaattctagaactctgagaggctgaagcaggaggattacttgtgaccaggagtttgagaccagcctgggcaacatagcaagaccttgtctctacagaaaataaaaaaaatagccaggtgtggtggtgtgcacctgtagtcttagctatgcgggtggcagaggcgggaggcttgcttcaggctggagtgagctatgatcatgtcacttacactccagcctgggtgagagagcaagaccctatctcaaaaaaaaaaaaagtgcaaactgaaaagttaatagcactttctcaaactgaattgacaccaacccaagagcgcgagaggaggatgacgactggcacctgtggaactgaactggaggctctgacttacggggtttttgcccccttctctatgaatgctggttccagctcagaaaagaccaacgcacgcgcttctgcagagtagccaggagagggcgcacaagacacgtgatggcaaaaaaacgaacaaagtctgaattttctctaaaaagaaaaaaaaagggggggagttcaccccatattactcttttttggaacaaagcaacataattttaccaaaatatatgctgagctttcaatcatcaaaacatattgatataatatttagttatgatttaccagtatgtataaagtccagttcataaattgtggtagatcttataaagcaaaataattaaatccctgtttggccactgagctgtgtgggattaggaaagttacttaacctctttgagttcttttcctcactgaaaaaaatggtaactatgataaccaccacagccaccaccacaccacaggttggctgagtgggtcagaatttggtctgagaagtaagtgatgtgtcacacgggaagtgcctgcacccagaggggctcagtcaaaaagggttccctttcctcattccctttactagatgtttttgtaaaaatctgtaggaaagcatttattaaaagcagcatcttcttaacaaacacaatgatgacatttaatattcccataggcttccttggattttggaatcaaacagagctgggttcaagtccaggcttcacatttcctagctgtgtgatctcaggcaaggtagctaccctctctgggcctttgtttccccctgtactatgaagccaattcccctgagtttcctgaggtggctgtgaggatgaaatgaggtggcacgcagcagggttgtcattaggagcatccgcttatggccgttctggccacaagacaagcaggagctgctgggaacagggcaagcagtgggtaccggcaaggagcggcatgacggccagctggatggagaaagcgctctgcttcctggggcctgtcagcgtggggtctgcctcttcttctgccaggggcttcttatgtctcctctggattttccttcttccctctgaatctttccctttaatttgagacctttgtctgtctaatatgtttgttaagctgctaagtgattcactctcaattaattccttgatctccatcatgcttgctcctgccaaagaaatggttggtgttcttgaaacactccattgaatcgtggaagaatcgtccattttgagggacttctcatattcctcactgttcttggaagaagtttcgggctctgcttggtgagaaccttgcaaagactttgggtgtttttctgttttttcttgttttcctggcggatgttcctggttcgactcttctctgacaatgttggtattctcaatgccctgttcagataattttctctgatttaaaaccaaatgtctcacttctgacttatgaaaagctcccacgtcgtctgtgaagccggcagtctttaatcggtaatatctgacttttcttgacatcttgtctttagtgttccagagcctcaaggtgattttgtggaaatttattttctttaataattcctttgtcacagtgatattaaaagtctgctcccacgacacccaggctttgtcaccttcgtgccacggcttcacagtctttactcctgactccaggaatactttggccaccattggaaatagcaatatgtcaacttttttaggttcttcatcgtccggcagaaggaaatactcaatgtggtaaaaacgacgcatctttgtaacagaactgtctgttttagggtgtttcttatatttttcaatcaaacttgcatattttcccttctgacccatattcacagggaaggccagtgagatggtgaatttgcaggggaccacgtggggcacgtcggagctgaaagtgctggcaggctcagatgaggactcgatgctgctgcacgggcggtcagagtcagactcctgggccctggccttggccttcaggtgttcctccacgtcacactcgctcgtggactggtaaaagctagtgatggaggagatgggctctatgcttgcggggtcctcttcccactcccaggcatgtagcgacatgctgcagagcgcactgctggccgccggcgctcctgcgagcggatgcgctgggcggcagcggggagttggaccgcggcggcaactcccgtaccggatccacagccacctgggcgaagagactccaagact

SEQ ID NO: 11269 - RNA, 5862 nt, Homo sapiens
  source 1..5862: mol_type = other RNA
ctgaatagctgggactacaggtgcccgacaacatgcctggctaattttttgtattgttagtaaagacggggtttcaccgtgttagccaggctgttctcgatctcctgacctcgtgatccacccgcctcggcctcccaaagtgtagggattacaggcgtgagccaccacacccagcccagaatgctttttctataaaaggtatccatgtatttcaccagtcagagatgtactaggtaaggaaaaaacaaaacaaataaacaaaaaaaatcacctcaagttttggaggcaggattgacctgggtttgaatcccagatctgactctttgtcatgtgataagctagagtctccaaggctcaatttcatcttcaaaatggggatagacaccaccttccttgggtttaaaggattaagaaagatgatatatgagatggtgctcaaaaagatcagtctattcctttcaacatgcctgtaaatgtatttctagggcatgtaaaagccaagtcgctcacattcagaaagagtaggcacttctaaaacaagtcccgggccaggtgtgcacagccatctgcacaggctgtgaacagaggcgtgcacagctcctgggggtagccctcatgctcccgcaggatcctctttaacaaagctgattcataaaagctgtcacccattacgcctgtgttctataattttgtgagccttttcacatgaaagactacccaagggtaggccgggtacggtggctcacgcctataatcccagcagtttggcaggccgaggcaggcggatcacctgaagtcgggagtttgagaccagcctgaccaaaatggagaaacctcgtctctaccaaaaatacaaaatcagccggacgtggtagcgcatgcctgtattcccaactactcaggaaggctaatgcaggagaatcgcttgaacccgggaggcggaggttgcggtgagctgagatcgcgccattgtactccagcctgggcaacaagagcaaaactccgtctcaaaaaaaaaaaaaagactactcaaggtagaaggaatccccattgcaaaaataaaaataaaaaaaaagtgctcaaatcatcagagtcagggagacatacaccagaacagaattccaggctgcgggctcacagcctccacactgctgacagttggggcagaccattctttgctcaggggacagtcctgtgcattatggcatgtttaacagtatcttactagatgccagtggcatcccactctcagtcgtgccaaccaaaatgcctccacacacagccaagtgtccccagcagacacaagccccctgagttaagagccctggttaagagtggaatggtgtaagggaatgtttgtgctcctccaacagccagtcccaaacatgcgctaatgtcatttcatccttaaccttgtgtggttgctgtcatctccacattacagatgggggaaatgaggcccagagttctgacgcaatcatccaaggtctcttagaaaatacgttgtagaaccagcatccaaaccagttctgttgggctaagtggggcccctccgctatgcaatactatccttttaaaataagagctcattcccagacacagaatctttctagaatcttactgggttactagccaaccaatatttactaataaggtatacatacatgatctatggcctaatttgaaattgaagatgattaccaaaaataattatgctgggcttacagtaaataatcttatgctattagtttctggcaaaaccagacatacaactggcctgctgagctgacccgttctctgtcgatgaccataggctatgtcatgggtataatggagcggcccacacacatggcctcaggacagctgctgcctccacacctgcaccccctgggtcccactgtgctagcagtttacacacgtcagctcctgtgatccttaaaacaacgctctgaggtaggagtaatcacccccatttcacagaggaggaaagtgagactcagagaaagtaggtaacttgctggtaagtggctgagccatgatcaaagtgttttggtcaccaaagttcttacatgtgaacccctgcactgtacagcattgtacatgacggggcaggttatagagaggggaggctaggtccagtgcggtagctcacgcctgtaatcccagcactttgggaggctgaggcaggtggatcactgtcaggcctctgagcccaagctaagccatcatatccccagtgacctgcatgtatacatccagatggcctgaagcaactgaagatccacaaaagaagtgaaaatagccttaactgatgacattccaccattgtgatttgtttctgccccaccctaactatcaatgtactttgtaatctcccccacacttaagaaggttctttataatctcccccacccttaagaaggtttttttgtaattctccccacccttgagaatgtactttgtgagatccaccccctgcccccaaaacattgctcttaactccactgcctatcccaaaacctgtaagaactaatgataatcccaccaccctttgctgactctcttttcagactcagcctgcctgcacccaggtgaaataaacagccttgttacttacacaaagcctgtttggtctcttcacacggacatgtaagacaatcacgaggtcaggagttcaagaccagcctggccaaaattgtgaaaccccatctctacaaaaaatacaaaaattagcctggcatggtggcatgcgcctgtaatcccagctactctagaggttgaagcaggagaattgcttaaacctgggggggcagaggctgtagtgagccgagatcgcgccactgcactccagcctgggcgacagagcaagactccatctcgaaaaaaaaaaaagagagaggggaccatgtcctggcttcattctgctggaaacagtcatgccaggcaggcccaaatggttgaacttctttttcctctcacagtaaaatccaaagcggggcaggtcccatggtacgctcccccaggaggatcatgggttcctccttgggactgtaggacgaaggaagcagctagcaaaggcgttcgctcaaagctactgtgtgcaataggtatgctggagggtcaggctggagcgtggggtggggtaagaccctctgaaagtttactctctgtcactgttgcctctcaagaggttctgatgctacgagaaagtgaaggtgatcaggaaggacaagctgtaggtgaagtatcattttcaaaaagtcatttaaaactgcaaactgccaaatgcggcagctcatgcctgtaattctagaactctgagaggctgaagcaggaggattacttgtgaccaggagtttgagaccagcctgggcaacatagcaagaccttgtctctacagaaaataaaaaaaatagccaggtgtggtggtgtgcacctgtagtcttagctatgcgggtggcagaggcgggaggcttgcttcaggctggagtgagctatgatcatgtcacttacactccagcctgggtgagagagcaagaccctatctcaaaaaaaaaaaaagtgcaaactgaaaagttaatagcactttctcaaactgaattgacaccaacccaagagcgcgagaggaggatgacgactggcacctgtggaactgaactggaggctctgacttacggggtttttgcccccttctctatgaatgctggttccagctcagaaaagaccaacgcacgcgcttctgcagagtagccaggagagggcgcacaagacacgtgatggcaaaaaaacgaacaaagtctgaattttctctaaaaagaaaaaaaaagggggggagttcaccccatattactcttttttggaacaaagcaacataattttaccaaaatatatgctgagctttcaatcatcaaaacatattgatataatatttagttatgatttaccagtatgtataaagtccagttcataaattgtggtagatcttataaagcaaaataattaaatccctgtttggccactgagctgtgtgggattaggaaagttacttaacctctttgagttcttttcctcactgaaaaaaatggtaactatgataaccaccacagccaccaccacaccacaggttggctgagtgggtcagaatttggtctgagaagtaagtgatgtgtcacacgggaagtgcctgcacccagaggggctcagtcaaaaagggttccctttcctcattccctttactagatgtttttgtaaaaatctgtaggaaagcatttattaaaagcagcatcttcttaacaaacacaatgatgacatttaatattcccataggcttccttggattttggaatcaaacagagctgggttcaagtccaggcttcacatttcctagctgtgtgatctcaggcaaggtagctaccctctctgggcctttgtttccccctgtactatgaagccaattcccctgagtttcctgaggtggctgtgaggatgaaatgaggtggcacgcagcagggttgtcattaggagcatccgcttatggccgttctggccacaagacaagcaggagctgctgggaacagggcaagcagtgggtaccggcaaggagcggcatgacggccagctggatggagaaagcgctctgcttcctggggcctgtcagcgtggggtctgcctcttcttctgccaggggcttcttatgtctcctctggattttccttcttccctctgaatctttccctttaatttgagacctttgtctgtctaatatgtttgttaagctgctaagtgattcactctcaattaattccttgatctccatcatgcttgctcctgccaaagaaatggttggtgttcttgaaacactccattgaatcgtggaagaatcgtccattttgagggacttctcatattcctcactgttcttggaagaagtttcgggctctgcttggtgagaaccttgcaaagactttgggtgtttttctgttttttcttgttttcctggcggatgttcctggttcgactcttctctgacaatgttggtattctcaatgccctgttcagataattttctctgatttaaaaccaaatgtctcacttctgacttatgaaaagctcccacgtcgtctgtgaagccggcagtctttaatcggtaatatctgacttttcttgacatcttgtctttagtgttccagagcctcaaggtgattttgtggaaatttattttctttaataattcctttgtcacagtgatattaaaagtctgctcccacgacacccaggctttgtcaccttcgtgccacggcttcacagtctttactcctgactccaggaatactttggccaccattggaaatagcaatatgtcaacttttttaggttcttcatcgtccggcagaaggaaatactcaatgtggtaaaaacgacgcatctttgtaacagaactgtctgttttagggtgtttcttatatttttcaatcaaacttgcatattttcccttctgacgtcagcagcgtgcaccagcaaaatagcagaagcaggaggagagccggctggaatacacctacccagagaagcaggtttttcttcatcttccagaaatgtgttctacggctacagggcggcgagagcaggcttgccaggcaaccctcgaaaggccttccgggaagagggggaagagtgacgcttgggtgtgggggcacatccccagcaaccggacgaggccgccacccccaaggccctcctgggcttcggatcccgcgccaacccctcgcccaggtctcggagcgaactctccgcgccaggcgggcggggcggagggaggagggagttgagagtggacggccgggagtgggaggaaaagcgcag

SEQ ID NO: 11270 - RNA, 5918 nt, Homo sapiens
  source 1..5918: mol_type = other RNA
ctgaatagctgggactacaggtgcccgacaacatgcctggctaattttttgtattgttagtaaagacggggtttcaccgtgttagccaggctgttctcgatctcctgacctcgtgatccacccgcctcggcctcccaaagtgtagggattacaggcgtgagccaccacacccagcccagaatgctttttctataaaaggtatccatgtatttcaccagtcagagatgtactaggtaaggaaaaaacaaaacaaataaacaaaaaaaatcacctcaagttttggaggcaggattgacctgggtttgaatcccagatctgactctttgtcatgtgataagctagagtctccaaggctcaatttcatcttcaaaatggggatagacaccaccttccttgggtttaaaggattaagaaagatgatatatgagatggtgctcaaaaagatcagtctattcctttcaacatgcctgtaaatgtatttctagggcatgtaaaagccaagtcgctcacattcagaaagagtaggcacttctaaaacaagtcccgggccaggtgtgcacagccatctgcacaggctgtgaacagaggcgtgcacagctcctgggggtagccctcatgctcccgcaggatcctctttaacaaagctgattcataaaagctgtcacccattacgcctgtgttctataattttgtgagccttttcacatgaaagactacccaagggtaggccgggtacggtggctcacgcctataatcccagcagtttggcaggccgaggcaggcggatcacctgaagtcgggagtttgagaccagcctgaccaaaatggagaaacctcgtctctaccaaaaatacaaaatcagccggacgtggtagcgcatgcctgtattcccaactactcaggaaggctaatgcaggagaatcgcttgaacccgggaggcggaggttgcggtgagctgagatcgcgccattgtactccagcctgggcaacaagagcaaaactccgtctcaaaaaaaaaaaaaagactactcaaggtagaaggaatccccattgcaaaaataaaaataaaaaaaaagtgctcaaatcatcagagtcagggagacatacaccagaacagaattccaggctgcgggctcacagcctccacactgctgacagttggggcagaccattctttgctcaggggacagtcctgtgcattatggcatgtttaacagtatcttactagatgccagtggcatcccactctcagtcgtgccaaccaaaatgcctccacacacagccaagtgtccccagcagacacaagccccctgagttaagagccctggttaagagtggaatggtgtaagggaatgtttgtgctcctccaacagccagtcccaaacatgcgctaatgtcatttcatccttaaccttgtgtggttgctgtcatctccacattacagatgggggaaatgaggcccagagttctgacgcaatcatccaaggtctcttagaaaatacgttgtagaaccagcatccaaaccagttctgttgggctaagtggggcccctccgctatgcaatactatccttttaaaataagagctcattcccagacacagaatctttctagaatcttactgggttactagccaaccaatatttactaataaggtatacatacatgatctatggcctaatttgaaattgaagatgattaccaaaaataattatgctgggcttacagtaaataatcttatgctattagtttctggcaaaaccagacatacaactggcctgctgagctgacccgttctctgtcgatgaccataggctatgtcatgggtataatggagcggcccacacacatggcctcaggacagctgctgcctccacacctgcaccccctgggtcccactgtgctagcagtttacacacgtcagctcctgtgatccttaaaacaacgctctgaggtaggagtaatcacccccatttcacagaggaggaaagtgagactcagagaaagtaggtaacttgctggtaagtggctgagccatgatcaaagtgttttggtcaccaaagttcttacatgtgaacccctgcactgtacagcattgtacatgacggggcaggttatagagaggggaggctaggtccagtgcggtagctcacgcctgtaatcccagcactttgggaggctgaggcaggtggatcactgtcaggcctctgagcccaagctaagccatcatatccccagtgacctgcatgtatacatccagatggcctgaagcaactgaagatccacaaaagaagtgaaaatagccttaactgatgacattccaccattgtgatttgtttctgccccaccctaactatcaatgtactttgtaatctcccccacacttaagaaggttctttataatctcccccacccttaagaaggtttttttgtaattctccccacccttgagaatgtactttgtgagatccaccccctgcccccaaaacattgctcttaactccactgcctatcccaaaacctgtaagaactaatgataatcccaccaccctttgctgactctcttttcagactcagcctgcctgcacccaggtgaaataaacagccttgttacttacacaaagcctgtttggtctcttcacacggacatgtaagacaatcacgaggtcaggagttcaagaccagcctggccaaaattgtgaaaccccatctctacaaaaaatacaaaaattagcctggcatggtggcatgcgcctgtaatcccagctactctagaggttgaagcaggagaattgcttaaacctgggggggcagaggctgtagtgagccgagatcgcgccactgcactccagcctgggcgacagagcaagactccatctcgaaaaaaaaaaaagagagaggggaccatgtcctggcttcattctgctggaaacagtcatgccaggcaggcccaaatggttgaacttctttttcctctcacagtaaaatccaaagcggggcaggtcccatggtacgctcccccaggaggatcatgggttcctccttgggactgtaggacgaaggaagcagctagcaaaggcgttcgctcaaagctactgtgtgcaataggtatgctggagggtcaggctggagcgtggggtggggtaagaccctctgaaagtttactctctgtcactgttgcctctcaagaggttctgatgctacgagaaagtgaaggtgatcaggaaggacaagctgtaggtgaagtatcattttcaaaaagtcatttaaaactgcaaactgccaaatgcggcagctcatgcctgtaattctagaactctgagaggctgaagcaggaggattacttgtgaccaggagtttgagaccagcctgggcaacatagcaagaccttgtctctacagaaaataaaaaaaatagccaggtgtggtggtgtgcacctgtagtcttagctatgcgggtggcagaggcgggaggcttgcttcaggctggagtgagctatgatcatgtcacttacactccagcctgggtgagagagcaagaccctatctcaaaaaaaaaaaaagtgcaaactgaaaagttaatagcactttctcaaactgaattgacaccaacccaagagcgcgagaggaggatgacgactggcacctgtggaactgaactggaggctctgacttacggggtttttgcccccttctctatgaatgctggttccagctcagaaaagaccaacgcacgcgcttctgcagagtagccaggagagggcgcacaagacacgtgatggcaaaaaaacgaacaaagtctgaattttctctaaaaagaaaaaaaaagggggggagttcaccccatattactcttttttggaacaaagcaacataattttaccaaaatatatgctgagctttcaatcatcaaaacatattgatataatatttagttatgatttaccagtatgtataaagtccagttcataaattgtggtagatcttataaagcaaaataattaaatccctgtttggccactgagctgtgtgggattaggaaagttacttaacctctttgagttcttttcctcactgaaaaaaatggtaactatgataaccaccacagccaccaccacaccacaggttggctgagtgggtcagaatttggtctgagaagtaagtgatgtgtcacacgggaagtgcctgcacccagaggggctcagtcaaaaagggttccctttcctcattccctttactagatgtttttgtaaaaatctgtaggaaagcatttattaaaagcagcatcttcttaacaaacacaatgatgacatttaatattcccataggcttccttggattttggaatcaaacagagctgggttcaagtccaggcttcacatttcctagctgtgtgatctcaggcaaggtagctaccctctctgggcctttgtttccccctgtactatgaagccaattcccctgagtttcctgaggtggctgtgaggatgaaatgaggtggcacgcagcagggttgtcattaggagcatccgcttatggccgttctggccacaagacaagcaggagctgctgggaacagggcaagcagtgggtaccggcaaggagcggcatgacggccagctggatggagaaagcgctctgcttcctggggcctgtcagcgtggggtctgcctcttcttctgccaggggcttcttatgtctcctctggattttccttcttccctctgaatctttccctttaatttgagacctttgtctgtctaatatgtttgttaagctgctaagtgattcactctcaattaattccttgatctccatcatgcttgctcctgccaaagaaatggttggtgttcttgaaacactccattgaatcgtggaagaatcgtccattttgagggacttctcatattcctcactgttcttggaagaagtttcgggctctgcttggtgagaaccttgcaaagactttgggtgtttttctgttttttcttgttttcctggcggatgttcctggttcgactcttctctgacaatgttggtattctcaatgccctgttcagataattttctctgatttaaaaccaaatgtctcacttctgacttatgaaaagctcccacgtcgtctgtgaagccggcagtctttaatcggtaatatctgacttttcttgacatcttgtctttagtgttccagagcctcaaggtgattttgtggaaatttattttctttaataattcctttgtcacagtgatattaaaagtctgctcccacgacacccaggctttgtcaccttcgtgccacggcttcacagtctttactcctgactccaggaatactttggccaccattggaaatagcaatatgtcaacttttttaggttcttcatcgtccggcagaaggaaatactcaatgtggtaaaaacgacgcatctttgtaacagaactgtctgttttagggtgtttcttatatttttcaatcaaacttgcatattttcccttctgacgtcagcagcgtgcaccagcaaaatagcagaagcaggaggagagccggctggaatacacctaccctggccggaagacatgaagatgagaaagaggccatccgggtacagcgtagcagttacgccagactaggacacttcctgtttacaggagactataaaacctttgccccgtcctcacttggggctgacgccattttaggcctcagccggcctgcaccaaggcgttcattgaaacagcatgttgctccacaccgcctcgtgttgtctgttggtgcgctctcggggttccaacccatacaagaaacttacaccatcgacagaataccaggagaagttgaaatcataatggtgggctagttcaagtaagcagatgaaaacaaaacaaagcaaggtctatcaagatgtgaagtactacttgt

SEQ ID NO: 11271 - RNA, 3808 nt, Homo sapiens
  source 1..3808: mol_type = other RNA
ctgaatagctgggactacaggtgcccgacaccacacccggctaattttttgtatttttagtagagacggggtttcactgtgttagccaggatggtctcgatctcctgacctcgtgatccacccacctcggcctcccaaagtgctgggattacaggcgtgagccactgcgcccggccacgacaggtagatttctcaatagggctgccttggtgtcttcatggcatgggaatgggcttttcccagtgtcagtatggtcaaagagagatcaaagaagaagccacagtgtattttgtgacctagccttggtcacttccaagcttttttggctataccaatggtgagagtggtactcattctcaacattgtgcaagtgcatgaccctgagtgtgaatacctccttaaattttttccctaggtgcattgattgcctccccttaatcctggcctcaggttacacaaatcatctgtattcagcattggaggggaccacataaagatgtgaatagtaggaggcaagaacactggggctcatcttggaggctggccaccacaagagttaagcacctacctaagattctgagccatgagaaagaacttccacaggctcgatggttctcaactttggctgaacatgtgaatcatttgagagtgttgatgcctgtgtctcactcctcagacattctgatttaattgaactgaagtgtgacagccatggtgtttaagaaaaagacataatctccaaataactctgcacaaggcattctcatgtgcagtcaaggataagcatactgcaagtgaactaaagtttccttttgggactaaagtccacacagaatttgcctatcactctatctgtcaacaacatctgtttttccctcctggagcagggagtgtgggaaggtttcaagcgacaaggaggattagtaatttattcattcacaaactattgctgaatacagagcacgtctggctgactaggtttcttctctgacacctatacattctgcttcaactgctttaaaaaagattggtaggagcagggttaattaatcagtgctggtctgatttgaggctctttatctttttcaaaacagatcaaaacaggcagattaaatgaacaggtaaatccccagatgaaaaagagaataactggaattagaaagtagggttgggcttaggctgcctgtttacttacaaaacagtttggttccagtttgatggacatacacacgaaggcactcaaatgaaaccactcttggctaatataattttagaggccagtggagttttgtatcttctaggctactgggtttttggctaattatctctttgatccctcttcatcctggtccatgtggcaggagtctgggctgaacatggtaggaagacagtgaaggaggattgaaaatgtggttcctgtgcaaagtattctgtttccttccatgaaaataagcaacagaatttcaatatgaagactaaccatacttctccattacttggcagccttgttagcacttttacattttctttttcctgtaattatcttagggaatgcagcaaagccccaggattttggcaaagagtttacaatgttgatagatgttcaaataagaggatcaggcatgggcatacagttgaaaccattgttgtccctccatcagagaatttaaatgaaaatactgtatttttttttaaagatggcagactaatatgtacttcttacataagcaagaaaaccactacgaattgcattgagtgtgaacatgacatatcctctcactcttggttaagcttcaggcgtttggagatggaagagggtgagttgctgggaaaacaggtcactcacttctgacttccatttcagctgcagcaaaggcatggctgaagagcgactatattaataaagcacaatgtctaccttctcaataggattccagcagagttctgccatggggcaaagtctcacgagactagagggtctccatctcatgataaggcagatcactttcgttgggctcttgaatgcaagtgtacttgatgggaggtggtggtggcttgaaaggtggaggtctttccattatttctttttggtactgacaccattttctcactccaagaccaaacaatatcatgcagcaaaagagtaaagctgctacaatcactggccaggacattccatctttgggcttattgaccacaataccagtgatatggacgtgattagttttcgtagatccattggcagttgtggggacttctgaaaatgctctggctgtgctggtaaagacattgtcatgaagtgttgagcctgcacctgacggggatgaactgtatgtttcactaggtatccgtgaaaattttttggtatctgtcccactggaggtccagggatagttgaagcctcgggtagtcatactggaattgctgggttgaggagtggtgtttggcctcaaggcactcacatctacaagggtcactgaagatgtagctggatatcttgcaggagatacactgctggctggagaaggttgggtgtcaagggtagattctgtaacactcagtggagggtctgttgaggaaatttcagaacctaagagaaaagtgatcttttctgatgagatgttccacactttatttcctgggactggagacagagccatacaccaaatggtcaagttgtctgattgggctggtttattactatgtacccttgttaaaacagacttcagttccaaaaatccatctttgccttttctctcttcattagtaatatatattccttctttttcatcatgaagaaaacttccatctataaaccatgtgatatttgctttgggaaatacattctttagtaagcaggtaaatcttctctctaccaagacatccgtggagttattttccacaatcacagggatttctggtttagcaaaaaccttgactgtggtggagctcctcaagattttgttaggaccgactctaatgtggcaagagaacttccgcccatcatcgaagatttggactggagagaggtggagtctgtagtctgtaccaagcttgactctatctttaagtaatgtggaattgctgatgaggtgattttgggagataagtgtttcctgagttccattatcctccaccgaccatgcataggtgaactcagatgaaatttttgaggagctattttgaaagcatggtatttccagagtctgatttatctctatttctatcgtatggttgctgttccattcatctgctgtaacgtgtgtctgaatgagaaggttgtagattttagtctgaatgccctctggatacagaacaagcatacactcgtaccttccactgactgaacaagacatattccttaagtgcagagtccattttgacccattctcaggagtttctgtgaaagtcacaagtgactcacagggtctcccataggcacagtagaagccgtattggggatgatagacagcaatcaggtctatcttattggtgaccttggaccattgcatctgcacgaagaagcctactgtctgtgtttggcaggtcaggttgacatcagagccaagtgtagcataaacattttcttctgtgttgactgttttttcccaaactcccttgacaaaatgtatctggatgatgtaatagacagcacagtatttccattttttctccattgtcttctgaacaccttacaccagcatttctgtaatgatcacaaagtcaattgatgttttcaagcaaactccagccacccacttcgtgctaaaaaacccgaactctaccacacacgcctgggtctgtttat

SEQ ID NO: 11272 - RNA, 3856 nt, Homo sapiens
  source 1..3856: mol_type = other RNA
ctgaatagctgggactacaggtgcccgacaccacacccggctaattttttgtatttttagtagagacggggtttcactgtgttagccaggatggtctcgatctcctgacctcgtgatccacccacctcggcctcccaaagtgctgggattacaggcgtgagccactgcgcccggccacgacaggtagatttctcaatagggctgccttggtgtcttcatggcatgggaatgggcttttcccagtgtcagtatggtcaaagagagatcaaagaagaagccacagtgtattttgtgacctagccttggtcacttccaagcttttttggctataccaatggtgagagtggtactcattctcaacattgtgcaagtgcatgaccctgagtgtgaatacctccttaaattttttccctaggtgcattgattgcctccccttaatcctggcctcaggttacacaaatcatctgtattcagcattggaggggaccacataaagatgtgaatagtaggaggcaagaacactggggctcatcttggaggctggccaccacaagagttaagcacctacctaagattctgagccatgagaaagaacttccacaggctcgatggttctcaactttggctgaacatgtgaatcatttgagagtgttgatgcctgtgtctcactcctcagacattctgatttaattgaactgaagtgtgacagccatggtgtttaagaaaaagacataatctccaaataactctgcacaaggcattctcatgtgcagtcaaggataagcatactgcaagtgaactaaagtttccttttgggactaaagtccacacagaatttgcctatcactctatctgtcaacaacatctgtttttccctcctggagcagggagtgtgggaaggtttcaagcgacaaggaggattagtaatttattcattcacaaactattgctgaatacagagcacgtctggctgactaggtttcttctctgacacctatacattctgcttcaactgctttaaaaaagattggtaggagcagggttaattaatcagtgctggtctgatttgaggctctttatctttttcaaaacagatcaaaacaggcagattaaatgaacaggtaaatccccagatgaaaaagagaataactggaattagaaagtagggttgggcttaggctgcctgtttacttacaaaacagtttggttccagtttgatggacatacacacgaaggcactcaaatgaaaccactcttggctaatataattttagaggccagtggagttttgtatcttctaggctactgggtttttggctaattatctctttgatccctcttcatcctggtccatgtggcaggagtctgggctgaacatggtaggaagacagtgaaggaggattgaaaatgtggttcctgtgcaaagtattctgtttccttccatgaaaataagcaacagaatttcaatatgaagactaaccatacttctccattacttggcagccttgttagcacttttacattttctttttcctgtaattatcttagggaatgcagcaaagccccaggattttggcaaagagtttacaatgttgatagatgttcaaataagaggatcaggcatgggcatacagttgaaaccattgttgtccctccatcagagaatttaaatgaaaatactgtatttttttttaaagatggcagactaatatgtacttcttacataagcaagaaaaccactacgaattgcattgagtgtgaacatgacatatcctctcactcttggttaagcttcaggcgtttggagatggaagagggtgagttgctgggaaaacaggtcactcacttctgacttccatttcagctgcagcaaaggcatggctgaagagcgactatattaataaagcacaatgtctaccttctcaataggattccagcagagttctgccatggggcaaagtctcacgagactagagggtctccatctcatgataaggcagatcactttcgttgggctcttgaatgcaagtgtacttgatgggaggtggtggtggcttgaaaggtggaggtctttccattatttctttttggtactgacaccattttctcactccaagaccaaacaatatcatgcagcaaaagagtaaagctgctacaatcactggccaggacattccatctttgggcttattgaccacaataccagtgatatggacgtgattagttttcgtagatccattggcagttgtggggacttctgaaaatgctctggctgtgctggtaaagacattgtcatgaagtgttgagcctgcacctgacggggatgaactgtatgtttcactaggtatccgtgaaaattttttggtatctgtcccactggaggtccagggatagttgaagcctcgggtagtcatactggaattgctgggttgaggagtggtgtttggcctcaaggcactcacatctacaagggtcactgaagatgtagctggatatcttgcaggagatacactgctggctggagaaggttgggtgtcaagggtagattctgtaacactcagtggagggtctgttgaggaaatttcagaacctaagagaaaagtgatcttttctgatgagatgttccacactttatttcctgggactggagacagagccatacaccaaatggtcaagttgtctgattgggctggtttattactatgtacccttgttaaaacagacttcagttccaaaaatccatctttgccttttctctcttcattagtaatatatattccttctttttcatcatgaagaaaacttccatctataaaccatgtgatatttgctttgggaaatacattctttagtaagcaggtaaatcttctctctaccaagacatccgtggagttattttccacaatcacagggatttctggtttagcaaaaaccttgactgtggtggagctcctcaagattttgttaggaccgactctaatgtggcaagagaacttccgcccatcatcgaagatttggactggagagaggtggagtctgtagtctgtaccaagcttgactctatctttaagtaatgtggaattgctgatgaggtgattttgggagataagtgtttcctgagttccattatcctcctttatacccttagaaagaaggacccaagaatccgtgctgctgttttccaccgaccatgcataggtgaactcagatgaaatttttgaggagctattttgaaagcatggtatttccagagtctgatttatctctatttctatcgtatggttgctgttccattcatctgctgtaacgtgtgtctgaatgagaaggttgtagattttagtctgaatgccctctggatacagaacaagcatacactcgtaccttccactgactgaacaagacatattccttaagtgcagagtccattttgacccattctcaggagtttctgtgaaagtcacaagtgactcacagggtctcccataggcacagtagaagccgtattggggatgatagacagcaatcaggtctatcttattggtgaccttggaccattgcatctgcacgaagaagcctactgtctgtgtttggcaggtcaggttgacatcagagccaagtgtagcataaacattttcttctgtgttgactgttttttcccaaactcccttgacaaaatgtatctggatgatgtaatagacagcacagtatttccattttttctccattgtcttctgaacaccttacaccagcatttctgtaatgatcacaaagtcaattgatgttttcaagcaaactccagccacccacttcgtgctaaaaaacccgaactctaccacacacgcctgggtctgtttat

SEQ ID NO: 11273 - RNA, 3547 nt, Homo sapiens
  source 1..3547: mol_type = other RNA
ctgaatagctgggactacaggtgcccgacaccacacccggctaattttttgtatttttagtagagacggggtttcactgtgttagccaggatggtctcgatctcctgacctcgtgatccacccacctcggcctcccaaagtgctgggattacaggcgtgagccactgcgcccggccacgacaggtagatttctcaatagggctgccttggtgtcttcatggcatgggaatgggcttttcccagtgtcagtatggtcaaagagagatcaaagaagaagccacagtgtattttgtgacctagccttggtcacttccaagcttttttggctataccaatggtgagagtggtactcattctcaacattgtgcaagtgcatgaccctgagtgtgaatacctccttaaattttttccctaggtgcattgattgcctccccttaatcctggcctcaggttacacaaatcatctgtattcagcattggaggggaccacataaagatgtgaatagtaggaggcaagaacactggggctcatcttggaggctggccaccacaagagttaagcacctacctaagattctgagccatgagaaagaacttccacaggctcgatggttctcaactttggctgaacatgtgaatcatttgagagtgttgatgcctgtgtctcactcctcagacattctgatttaattgaactgaagtgtgacagccatggtgtttaagaaaaagacataatctccaaataactctgcacaaggcattctcatgtgcagtcaaggataagcatactgcaagtgaactaaagtttccttttgggactaaagtccacacagaatttgcctatcactctatctgtcaacaacatctgtttttccctcctggagcagggagtgtgggaaggtttcaagcgacaaggaggattagtaatttattcattcacaaactattgctgaatacagagcacgtctggctgactaggtttcttctctgacacctatacattctgcttcaactgctttaaaaaagattggtaggagcagggttaattaatcagtgctggtctgatttgaggctctttatctttttcaaaacagatcaaaacaggcagattaaatgaacaggtaaatccccagatgaaaaagagaataactggaattagaaagtagggttgggcttaggctgcctgtttacttacaaaacagtttggttccagtttgatggacatacacacgaaggcactcaaatgaaaccactcttggctaatataattttagaggccagtggagttttgtatcttctaggctactgggtttttggctaattatctctttgatccctcttcatcctggtccatgtggcaggagtctgggctgaacatggtaggaagacagtgaaggaggattgaaaatgtggttcctgtgcaaagtattctgtttccttccatgaaaataagcaacagaatttcaatatgaagactaaccatacttctccattacttggcagccttgttagcacttttacattttctttttcctgtaattatcttagggaatgcagcaaagccccaggattttggcaaagagtttacaatgttgatagatgttcaaataagaggatcaggcatgggcatacagttgaaaccattgttgtccctccatcagagaatttaaatgaaaatactgtatttttttttaaagatggcagactaatatgtacttcttacataagcaagaaaaccactacgaattgcattgagtgtgaacatgacatatcctctcactcttggttaagcttcaggcgtttggagatggaagagggtgagttgctgggaaaacaggtcactcacttctgacttccatttcagctgcagcaaaggcatggctgaagagcgactatattaataaagcacaatgtctaccttctcaataggattccagcagagttctgccatggggcaaagtctcacgagactagagggtctccatctcatgataaggcagatcactttcgttgggctcttgaatgcaagtgtacttgatgggaggtggtggtggcttgaaaggtggaggtctttccattatttctttttggtactgacaccattttctcactccaagaccaaacaatatcatgcagcaaaagagtaaagctgctacaatcactggccaggacattccatctttgggcttattgaccacaataccagtgatatggacgtgattagttttcgtagatccattggcagttgtggggacttctgaaaatgctctggctgtgctggtaaagacattgtcatgaagtgttgagcctgcacctgacggggatgaactgtatgtttcactaggtatccgtgaaactgattttttggtatctgtcccactggaggtccagggatagttgaagcctcgggtagtcatactggaattgctgggttgaggagtggtgtttggcctcaaggcactcacatctacaagggtcactgaagatgtagctggatatcttgcaggagatacactgctggctggagaaggttgggtgtcaagggtagattctgtaacactcagtggagggtctgttgaggaaatttcagaacctaagagaaaagtgatcttttctgatgagatgttccacactttatttcctgggactggagacagagccatacaccaaatggtcaagttgtctgattgggctggtttattactatgtacccttgttaaaacagacttcagttccaaaaatccatctttgccttttctctcttcattagtaatatatattccttctttttcatcatgaagaaaacttccatctataaaccatgtgatatttgctttgggaaatacattctttagtaagcaggtaaatcttctcaccgaccatgcataggtgaactcagatgaaatttttgaggagctattttgaaagcatggtatttccagagtctgatttatctctatttctatcgtatggttgctgttccattcatctgctgtaacgtgtgtctgaatgagaaggttgtagattttagtctgaatgccctctggatacagaacaagcatacactcgtaccttccactgactgaacaagacatattccttaagtgcagagtccattttgacccattctcaggagtttctgtgaaagtcacaagtgactcacagggtctcccataggcacagtagaagccgtattggggatgatagacagcaatcaggtctatcttattggtgaccttggaccattgcatctgcacgaagaagcctactgtctgtgtttggcaggtcaggttgacatcagagccaagtgtagcataaacattttcttctgtgttgactgttttttcccaaactcccttgacaaaatgtatctggatgatgtaatagacagcacagtatttccattttttctccattgtcttctgaacaccttacaccagcatttctgtaatgatcacaaagtcaattgatgttttcaagcaaactccagccacccacttcgtgctaaaaaacccgaactctaccacacacgcctgggtctgtttat

SEQ ID NO: 11274 - RNA, 3732 nt, Homo sapiens
  source 1..3732: mol_type = other RNA
ctgaatagctgggactacaggtgcccgacaccacacccggctaattttttgtatttttagtagagacggggtttcactgtgttagccaggatggtctcgatctcctgacctcgtgatccacccacctcggcctcccaaagtgctgggattacaggcgtgagccactgcgcccggccacgacaggtagatttctcaatagggctgccttggtgtcttcatggcatgggaatgggcttttcccagtgtcagtatggtcaaagagagatcaaagaagaagccacagtgtattttgtgacctagccttggtcacttccaagcttttttggctataccaatggtgagagtggtactcattctcaacattgtgcaagtgcatgaccctgagtgtgaatacctccttaaattttttccctaggtgcattgattgcctccccttaatcctggcctcaggttacacaaatcatctgtattcagcattggaggggaccacataaagatgtgaatagtaggaggcaagaacactggggctcatcttggaggctggccaccacaagagttaagcacctacctaagattctgagccatgagaaagaacttccacaggctcgatggttctcaactttggctgaacatgtgaatcatttgagagtgttgatgcctgtgtctcactcctcagacattctgatttaattgaactgaagtgtgacagccatggtgtttaagaaaaagacataatctccaaataactctgcacaaggcattctcatgtgcagtcaaggataagcatactgcaagtgaactaaagtttccttttgggactaaagtccacacagaatttgcctatcactctatctgtcaacaacatctgtttttccctcctggagcagggagtgtgggaaggtttcaagcgacaaggaggattagtaatttattcattcacaaactattgctgaatacagagcacgtctggctgactaggtttcttctctgacacctatacattctgcttcaactgctttaaaaaagattggtaggagcagggttaattaatcagtgctggtctgatttgaggctctttatctttttcaaaacagatcaaaacaggcagattaaatgaacaggtaaatccccagatgaaaaagagaataactggaattagaaagtagggttgggcttaggctgcctgtttacttacaaaacagtttggttccagtttgatggacatacacacgaaggcactcaaatgaaaccactcttggctaatataattttagaggccagtggagttttgtatcttctaggctactgggtttttggctaattatctctttgatccctcttcatcctggtccatgtggcaggagtctgggctgaacatggtaggaagacagtgaaggaggattgaaaatgtggttcctgtgcaaagtattctgtttccttccatgaaaataagcaacagaatttcaatatgaagactaaccatacttctccattacttggcagccttgttagcacttttacattttctttttcctgtaattatcttagggaatgcagcaaagccccaggattttggcaaagagtttacaatgttgatagatgttcaaataagaggatcaggcatgggcatacagttgaaaccattgttgtccctccatcagagaatttaaatgaaaatactgtatttttttttaaagatggcagactaatatgtacttcttacataagcaagaaaaccactacgaattgcattgagtgtgaacatgacatatcctctcactcttggttaagcttcaggcgtttggagatggaagagggtgagttgctgggaaaacaggtcactcacttctgacttccatttcagctgcagcaaaggcatggctgaagagcgactatattaataaagcacaatgtctaccttctcaataggattccagcagagttctgccatggggcaaagtctcacgagactagagggtctccatctcatgataaggcagatcactttcgttgggctcttgaatgcaagtgtacttgatgggaggtggtggtggcttgaaaggtggaggtctttccattatttctttttggtactgacaccattttctcactccaagaccaaacaatatcatgcagcaaaagagtaaagctgctacaatcactggccaggacattccatctttgggcttattgaccacaataccagtgatatggacgtgattagttttcgtagatccattggcagttgtggggacttctgaaaatgctctggctgtgctggtaaagacattgtcatgaagtgttgagcctgcacctgacggggatgaactgtatgtttcactaggtatccgtgaaactgattttttggtatctgtcccactggaggtccagggatagttgaagcctcgggtagtcatactggaattgctgggttgaggagtggtgtttggcctcaaggcactcacatctacaagggtcactgaagatgtagctggatatcttgcaggagatacactgctggctggagaaggttgggtgtcaagggtagattctgtaacactcagtggagggtctgttgaggaaatttcagaacctaagagaaaagtgatcttttctgatgagatgttccacactttatttcctgggactggagacagagccatacaccaaatggtcaagttgtctgattgggctggtttattactatgtacccttgttaaaacagacttcagttccaaaaatccatctttgccttttctctcttcattagtaatatatattccttctttttcatcatgaagaaaacttccatctataaaccatgtgatatttgctttgggaaatacattctttagtaagcaggtaaatcttctctctaccaagacatccgtggagttattttccacaatcacagggatttctggtttagcaaaaaccttgactgtggtggagctcctcaagattttgttaggaccgactctaatgtggcaagagaacttccgcccatcatcgaagatttggactggagagaggtggagtctgtagtctgtaccaagcttgactctatctttaagtaatgtggaattgctgatgaggtgattttgggagataagtgtttcctgagttccattatcctccaccgaccatgcataggtgaactcagatgaaatttttgaggagctattttgaaagcatggtatttccagagtctgatttatctctatttctatcgtatggttgctgttccattcatctgctgtaacgtgtgtctgaatgagaaggttgtagattttagtctgaatgccctctggatacagaacaagcatacactcgtaccttccactgactgaacaagacatattccttaagtgcagagtccattttgacccattctcaggagtttctgtgaaagtcacaagtgactcacagggtctcccataggcacagtagaagccgtattggggatgatagacagcaatcaggtctatcttattggtgaccttggaccattgcatctgcacgaagaagcctactgtctgtgtttggcaggtcaggttgacatcagagccaagtgtagcataaacattttcttctgtgttgactgttttttcccaaactcccttgacaaaatgtatctggatgatgtaatagacagcacagtatttccattttttctccattgtcttctgaacaccttacaccagcatttctgtaatgatcacaaagtcaatt

SEQ ID NO: 11275 - RNA, 3780 nt, Homo sapiens
  source 1..3780: mol_type = other RNA
ctgaatagctgggactacaggtgcccgacaccacacccggctaattttttgtatttttagtagagacggggtttcactgtgttagccaggatggtctcgatctcctgacctcgtgatccacccacctcggcctcccaaagtgctgggattacaggcgtgagccactgcgcccggccacgacaggtagatttctcaatagggctgccttggtgtcttcatggcatgggaatgggcttttcccagtgtcagtatggtcaaagagagatcaaagaagaagccacagtgtattttgtgacctagccttggtcacttccaagcttttttggctataccaatggtgagagtggtactcattctcaacattgtgcaagtgcatgaccctgagtgtgaatacctccttaaattttttccctaggtgcattgattgcctccccttaatcctggcctcaggttacacaaatcatctgtattcagcattggaggggaccacataaagatgtgaatagtaggaggcaagaacactggggctcatcttggaggctggccaccacaagagttaagcacctacctaagattctgagccatgagaaagaacttccacaggctcgatggttctcaactttggctgaacatgtgaatcatttgagagtgttgatgcctgtgtctcactcctcagacattctgatttaattgaactgaagtgtgacagccatggtgtttaagaaaaagacataatctccaaataactctgcacaaggcattctcatgtgcagtcaaggataagcatactgcaagtgaactaaagtttccttttgggactaaagtccacacagaatttgcctatcactctatctgtcaacaacatctgtttttccctcctggagcagggagtgtgggaaggtttcaagcgacaaggaggattagtaatttattcattcacaaactattgctgaatacagagcacgtctggctgactaggtttcttctctgacacctatacattctgcttcaactgctttaaaaaagattggtaggagcagggttaattaatcagtgctggtctgatttgaggctctttatctttttcaaaacagatcaaaacaggcagattaaatgaacaggtaaatccccagatgaaaaagagaataactggaattagaaagtagggttgggcttaggctgcctgtttacttacaaaacagtttggttccagtttgatggacatacacacgaaggcactcaaatgaaaccactcttggctaatataattttagaggccagtggagttttgtatcttctaggctactgggtttttggctaattatctctttgatccctcttcatcctggtccatgtggcaggagtctgggctgaacatggtaggaagacagtgaaggaggattgaaaatgtggttcctgtgcaaagtattctgtttccttccatgaaaataagcaacagaatttcaatatgaagactaaccatacttctccattacttggcagccttgttagcacttttacattttctttttcctgtaattatcttagggaatgcagcaaagccccaggattttggcaaagagtttacaatgttgatagatgttcaaataagaggatcaggcatgggcatacagttgaaaccattgttgtccctccatcagagaatttaaatgaaaatactgtatttttttttaaagatggcagactaatatgtacttcttacataagcaagaaaaccactacgaattgcattgagtgtgaacatgacatatcctctcactcttggttaagcttcaggcgtttggagatggaagagggtgagttgctgggaaaacaggtcactcacttctgacttccatttcagctgcagcaaaggcatggctgaagagcgactatattaataaagcacaatgtctaccttctcaataggattccagcagagttctgccatggggcaaagtctcacgagactagagggtctccatctcatgataaggcagatcactttcgttgggctcttgaatgcaagtgtacttgatgggaggtggtggtggcttgaaaggtggaggtctttccattatttctttttggtactgacaccattttctcactccaagaccaaacaatatcatgcagcaaaagagtaaagctgctacaatcactggccaggacattccatctttgggcttattgaccacaataccagtgatatggacgtgattagttttcgtagatccattggcagttgtggggacttctgaaaatgctctggctgtgctggtaaagacattgtcatgaagtgttgagcctgcacctgacggggatgaactgtatgtttcactaggtatccgtgaaactgattttttggtatctgtcccactggaggtccagggatagttgaagcctcgggtagtcatactggaattgctgggttgaggagtggtgtttggcctcaaggcactcacatctacaagggtcactgaagatgtagctggatatcttgcaggagatacactgctggctggagaaggttgggtgtcaagggtagattctgtaacactcagtggagggtctgttgaggaaatttcagaacctaagagaaaagtgatcttttctgatgagatgttccacactttatttcctgggactggagacagagccatacaccaaatggtcaagttgtctgattgggctggtttattactatgtacccttgttaaaacagacttcagttccaaaaatccatctttgccttttctctcttcattagtaatatatattccttctttttcatcatgaagaaaacttccatctataaaccatgtgatatttgctttgggaaatacattctttagtaagcaggtaaatcttctctctaccaagacatccgtggagttattttccacaatcacagggatttctggtttagcaaaaaccttgactgtggtggagctcctcaagattttgttaggaccgactctaatgtggcaagagaacttccgcccatcatcgaagatttggactggagagaggtggagtctgtagtctgtaccaagcttgactctatctttaagtaatgtggaattgctgatgaggtgattttgggagataagtgtttcctgagttccattatcctcctttatacccttagaaagaaggacccaagaatccgtgctgctgttttccaccgaccatgcataggtgaactcagatgaaatttttgaggagctattttgaaagcatggtatttccagagtctgatttatctctatttctatcgtatggttgctgttccattcatctgctgtaacgtgtgtctgaatgagaaggttgtagattttagtctgaatgccctctggatacagaacaagcatacactcgtaccttccactgactgaacaagacatattccttaagtgcagagtccattttgacccattctcaggagtttctgtgaaagtcacaagtgactcacagggtctcccataggcacagtagaagccgtattggggatgatagacagcaatcaggtctatcttattggtgaccttggaccattgcatctgcacgaagaagcctactgtctgtgtttggcaggtcaggttgacatcagagccaagtgtagcataaacattttcttctgtgttgactgttttttcccaaactcccttgacaaaatgtatctggatgatgtaatagacagcacagtatttccattttttctccattgtcttctgaacaccttacaccagcatttctgtaatgatcacaaagtcaatt

SEQ ID NO: 11276 - RNA, 3670 nt, Homo sapiens
  source 1..3670: mol_type = other RNA
ctgaatagctgggactacaggtgcccgacaccacacccggctaattttttgtatttttagtagagacggggtttcactgtgttagccaggatggtctcgatctcctgacctcgtgatccacccacctcggcctcccaaagtgctgggattacaggcgtgagccactgcgcccggccacgacaggtagatttctcaatagggctgccttggtgtcttcatggcatgggaatgggcttttcccagtgtcagtatggtcaaagagagatcaaagaagaagccacagtgtattttgtgacctagccttggtcacttccaagcttttttggctataccaatggtgagagtggtactcattctcaacattgtgcaagtgcatgaccctgagtgtgaatacctccttaaattttttccctaggtgcattgattgcctccccttaatcctggcctcaggttacacaaatcatctgtattcagcattggaggggaccacataaagatgtgaatagtaggaggcaagaacactggggctcatcttggaggctggccaccacaagagttaagcacctacctaagattctgagccatgagaaagaacttccacaggctcgatggttctcaactttggctgaacatgtgaatcatttgagagtgttgatgcctgtgtctcactcctcagacattctgatttaattgaactgaagtgtgacagccatggtgtttaagaaaaagacataatctccaaataactctgcacaaggcattctcatgtgcagtcaaggataagcatactgcaagtgaactaaagtttccttttgggactaaagtccacacagaatttgcctatcactctatctgtcaacaacatctgtttttccctcctggagcagggagtgtgggaaggtttcaagcgacaaggaggattagtaatttattcattcacaaactattgctgaatacagagcacgtctggctgactaggtttcttctctgacacctatacattctgcttcaactgctttaaaaaagattggtaggagcagggttaattaatcagtgctggtctgatttgaggctctttatctttttcaaaacagatcaaaacaggcagattaaatgaacaggtaaatccccagatgaaaaagagaataactggaattagaaagtagggttgggcttaggctgcctgtttacttacaaaacagtttggttccagtttgatggacatacacacgaaggcactcaaatgaaaccactcttggctaatataattttagaggccagtggagttttgtatcttctaggctactgggtttttggctaattatctctttgatccctcttcatcctggtccatgtggcaggagtctgggctgaacatggtaggaagacagtgaaggaggattgaaaatgtggttcctgtgcaaagtattctgtttccttccatgaaaataagcaacagaatttcaatatgaagactaaccatacttctccattacttggcagccttgttagcacttttacattttctttttcctgtaattatcttagggaatgcagcaaagccccaggattttggcaaagagtttacaatgttgatagatgttcaaataagaggatcaggcatgggcatacagttgaaaccattgttgtccctccatcagagaatttaaatgaaaatactgtatttttttttaaagatggcagactaatatgtacttcttacataagcaagaaaaccactacgaattgcattgagtgtgaacatgacatatcctctcactcttggttaagcttcaggcgtttggagatggaagagggtgagttgctgggaaaacaggtcactcacttctgacttccatttcagctgcagcaaaggcatggctgaagagcgactatattaataaagcacaatgtctaccttctcaataggattccagcagagttctgccatggggcaaagtctcacgagactagagggtctccatctcatgataaggcagatcactttcgttgggctcttgaatgcaagtgtacttgatgggaggtggtggtggcttgaaaggtggaggtctttccattatttctttttggtactgacaccattttctcactccaagaccaaacaatatcatgcagcaaaagagtaaagctgctacaatcactggccaggacattccatctttgggcttattgaccacaataccagtgatatggacgtgattagttttcgtagatccattggcagttgtggggacttctgaaaatgctctggctgtgctggtaaagacattgtcatgaagtgttgagcctgcacctgacggggatgaactgtatgtttcactaggtatccgtgaaactgattttttggtatctgtcccactggaggtccagggatagttgaagcctcgggtagtcatactggaattgctgggttgaggagtggtgtttggcctcaaggcactcacatctacaagggtcactgaagatgtagctggatatcttgcaggagatacactgctggctggagaaggttgggtgtcaagggtagattctgtaacactcagtggagggtctgttgaggaaatttcagaaccttctttttcatcatgaagaaaacttccatctataaaccatgtgatatttgctttgggaaatacattctttagtaagcaggtaaatcttctctctaccaagacatccgtggagttattttccacaatcacagggatttctggtttagcaaaaaccttgactgtggtggagctcctcaagattttgttaggaccgactctaatgtggcaagagaacttccgcccatcatcgaagatttggactggagagaggtggagtctgtagtctgtaccaagcttgactctatctttaagtaatgtggaattgctgatgaggtgattttgggagataagtgtttcctgagttccattatcctcctttatacccttagaaagaaggacccaagaatccgtgctgctgttttccaccgaccatgcataggtgaactcagatgaaatttttgaggagctattttgaaagcatggtatttccagagtctgatttatctctatttctatcgtatggttgctgttccattcatctgctgtaacgtgtgtctgaatgagaaggttgtagattttagtctgaatgccctctggatacagaacaagcatacactcgtaccttccactgactgaacaagacatattccttaagtgcagagtccattttgacccattctcaggagtttctgtgaaagtcacaagtgactcacagggtctcccataggcacagtagaagccgtattggggatgatagacagcaatcaggtctatcttattggtgaccttggaccattgcatctgcacgaagaagcctactgtctgtgtttggcaggtcaggttgacatcagagccaagtgtagcataaacattttcttctgtgttgactgttttttcccaaactcccttgacaaaatgtatctggatgatgtaatagacagcacagtatttccattttttctccattgtcttctgaacaccttacaccagcatttctgtaatgatcacaaagtcaattgatgttttcaagcaaactccagccacccacttcgtgctaaaaaacccgaactctaccacacacgcctgggtctgtttat

SEQ ID NO: 11277 - RNA, 1382 nt, Homo sapiens
  source 1..1382: mol_type = other RNA
ctgaatagctgggactacaggtgcccgccaacacgcccaggtaattttttgtattcgtagtagagacggggtttcaccgtgttagccaggatggtcttgatctcctgacctcgtgatctgcccgtctcggcctcccaaagtgccgggattacaggtatgagcccccgcgcccggccaacatgactctttagaagtcaatcctgaatgtcaaaaatatgctgtttagggtttagaatcaacatactttcttcctgtgccacaaccacacacgcagggaagacctcaccctgtggaaatacggtcctctgctgcccactgcatcagagttgatgccgggacaataaactcctacaggaagaacaagtgagcttttggcccctttcttcagaacccgctcccctcctggagaagcccacacacacactgcagcagtggggagctgggctggactaagctccccttcagggcacagacctggctctgaccaaaccccatgcagagcacagcaccccctcacctctttgtgaatcagaggctgaactcagccttcagaaatgagaacacggcttcggtgctcaatgctggatacagaatacagtaaaatccctttatccaaggggatacgttgcaaaaccctgagtgaatgaaacttggaacagtactgaaccctatttactccacttaaaggatgcctgtgacagattctcactgacatatccaaattgccaacatcaatgctcatgtgcttggggggcatgttaagtaaaataaggatcacttaaacaaaaccaatgaggtaccacaaaattggatctgatcaaaaagactactattaaaaacaaaacaaaacaaaacaaaaaagaagactattaacagattgatgggcagacagagtatacagtgcatggggtctgtatccatggattcaaccaattacagacttaaataatttaaaaaagacaaaaggaagcaatataccaatataaaatagcaatacaataaaaataatacaagaaaacaacccagtataacaagcatttacatagcatttatatttaattaggtattaccagtaatcagatgtttacagtatatgggagggtgcagaggatgtgcataggttacatgcaaatgcagtcacgcatcgcttaataacagggacatgttctgagaaacgcattttcagaccatttcattacagagggaacttacacaaaccaagatagcatagcctactacacatctggtatatataatacagcctactgctaaaaacctgtagggcatgctatgtcctgaatactatagtcaactgtaacaacggtaagtactcgtaagtcaaaacatatctaaatatagaaaaggtacagtaaggccaggca

SEQ ID NO: 11278 - RNA, 4567 nt, Homo sapiens
  source 1..4567: mol_type = other RNA
ctgaatagctgggactacaggtgcccgccaacatgtccggctaattttttgtatttttagtagagatggggtttcaccatgttagccaggatggtcttgatctcctgacctcatgatccgcccacctcagcctcccaaagttctgggattacaggcatgagccactgtgcccggcctaattttcgtatttttagtagagagggggtttcaccatgttggtcaggatggtctcgatctactgaccttgtgatctgcccgcctcggcctcccaaagtgctgggaatacaggtgtgagccaccatgcgcagcctgctgttactttcagtggcaaaaccacaattacttctgcacctaccttgtaggggtgttgcttaacacttattgagattgtgcatataaaggagttagcattgttcagataataaatctcggttgtcatcatcattattgtcatcatgctgatacccagtaagtgaatccatgcaatctaaatccttcatccttttctccagttctagcccagggtcccttggccagaacacatggtcaattgtaaacttgagaggatgtactgggacactttgtaggttttgtaggttgctgacatttcttaaactaactgcatttgttttctagcaatgttgcaacaaagtaccacaaatcaggccgagtgtggtggtttacacctgcaatcccagcactttgtgaagccgaggagggcagatctcttgaggccgggagtttgagaccagcctgggcaacatagtgagaccctgtctctacaaatatatatagctgattgcagtggcataggcctgtagtcccaactactcaggaggctgaggcaggaggattgcttgagcccaggagtttgaggtgaggttgcactttagctatgattgcaccactgtactccagcctgggtgacacagtagatcctgtctgtctctaaaagaaaaaaaaatttaaaaattaccatgaactaggtgacttaaacaatagaaatttgttgtcttacagttctggaggttaagagtccgagatcaaggtgttgggccaggtgcagtggcccacgcttgtaatcccagcactttgggaggctgaggtgggcagatcactggaggccaggagtttgagaccagtctggccaacatagtgaaatcccatctctactaaaaacacaaaattagctgggcgtggtggtgggtgcctgtaatcccagctacttgggaggctgaggcaggagaattgcttgaacctgggaggtggaggttgcagtgagccaaaatcatgccactgcatccagccgggatgacagagcaagactccgtctcaaaaaaaaaaaaaaaaaaaaaagatcagttgtcagcagctttgattccttggttccttctgagggctgagagggatagcctgttccacgcctctcctggcttctggtggtctgcaggcagtccctggcattccttggcttgtaggagcatcaccccaatctctgcctccatcttcatgtggcggtctccatgtgtgtgggtgcctgtgtccaaatctccccttttcataaggacgccagtcgtatcagattagggaccaacctaatgaccttactgtaatctaatgacctctgtaaacaccctatcttcaaatatggtcacattctgaggtccttggggttaggacttcaacatatcttttttattttattattattacttttgcagacagggccttgctctgtttcccaggctggagtgcagtggcaggaacatagctcatgcagcctcgacctccttggctcaagaggtcctcctgtctcagcctcccgagtaactaagatgacaggtgcacaccaccacacccaggtaattttttcttttttcatttttattttttgtagggatgagatctcactatgttgttcaggctggtcctgaactcctagcttcaaatgattctccctactcaacctcccaaagtgccagagtttacaggtgtgagccactgcgcctggcctcccacgtatctttttttgggagccacagttcaacccataacactaactttttaagtgccccgggccacctgatctgctgtggctgaccctgcgtgtagaatcatactgggttcagagtcaggcgatgaatgtcacaggaaacacatagattttggagctaggctagggtctgtgttcccaaactacgattgatggaccgtctgcatcagagtccccttgactgggggttgtggggagacaggaagcctgttgggaattgagaaagtaagccccaaccacagtcatagttacaagtggaggtctcaagaccccccaggaggctgaggcttgctggctgactaagcgaacagcacgtgagctaatctcacttgcaaatattttcaaagttcttccacaacacttaggaaacactggctaatacatgggctgtctgtatctacctatctatctatctatctatctacctacctcctctatctctatctatccatccatctatctatcatctatctgttgatcgattgatcaatcgatcgactgacctacctacctatctcatctatctatctatctatctatctatctatcatctatctacttatatgatctatctatcaatcaatcatctatctgtctgtcaatagatagatctatcgatcggttgacctacctacctacctacctatctatcctatctatctatgtatctatctgtatatctatctatctatctatctatctatctatctatctatctatctatctacatatcttatctatccaccctatctacctatcttatcttatcctctctatctatctgtctgtctatctatctatctatctatctatctatctatctatctatctatctacctatgagtgacagatcttgctcagtttcccaaactgctgaagtgcagtggtgcagtcatagctcactgcaaccttgaactcctgggctcaaatgatctgcctgcctcagcctcctgattagctgagactacaggcgtataccaccatgtcttgctaaagtgattttgtgtgtgtgtgtggagatagggtctctgtatgttgcccaggctggtctcaaactcctggcctcaagtgatccttccaccttggcctcccaaaatgctgggatcacaggcttgagcttccacacctggcctttgtcaatactaaaatgagtgtagctacgtctcttgttttcaactactcttattcacatagcaatcctaaaaggctgatcctccaggagggctaatttcaggccagtttgatccttgctattctgatctttttggggaagataaatcctggggaaaatgcacacctttcctttgggtgctcatacactttgttcatctctttatgacacatttatcacgttgtactggaaggatttattccatgtctctgttcccagctagactctgaactcctccagggtaggggatgggatgcatctctgtgtccctagcagccaacagtgatcctggaacatgataaacatccaataactgttctggcctaggacaggggacggccactttgccgatgagcttccccagggctgccttcatatccttgttccgtatgctgtagataaaggggttgagcatggggatgaacaccccacacattagggcggctgccttgtccttctgggaggagctgggggatgtgggctgtaagtacacagcaaagatggtcccataggacagtgacaccacagtgaggtgtaagccacaggtggagaaggctttccacttgccccgagtagaagggatcttaaagactgtccagaaaatgcggatgtacgagagaaggatgcaggagaatgggctggtgcccacgacaatgccaaaagcaaagatcaccagctcgttggtgtgcgtgtctgagccggagagcttcagcaggggcatgaggtcacagaagaagtgggagatttcagagccggcgcagaaggtcagttgagccatgaggcaggtgtgtatgagagactggaggttggtgatcatccatgatgctcccagcagcagcccacagacaggggagcacatgagaaccaagtaacgctgtgggtggacaatggccacgaagcggtcgatggccattactgccaggagaaagctgtccatggtcccgaacaggtggaaggcatacatctgggtgaggcagcccacaaaggggatggctctgctctgagcctggatgttcgctagcatcttggggacggtggtggaggataatagggtgtcaacgagtgagaggttgaagagaaagaagtacatgggtgtgtggaggtgagagtccgtgatgatggccaggataatgagggcatttccaatgatggtgaccaggtatgtggagaggaacattgtgaagaggagggtctgatgctctggcttttctgagagtccctggaggaagaattctgagatttcggtttgcttttctggttccatgtatggtctgtgactgtgatcgctggggttagcctgatgtctatgggaaggattcatatgtgtacccccccgcccccag

SEQ ID NO: 11279 - RNA, 178 nt, Homo sapiens
  source 1..178: mol_type = other RNA
ctgaatagctgggactacaggtgcccgccaccacacccagctaatttttttgtattttagtagagatggggtttcatcttgcccaagctggttgggaactcctgagctcaggcaatctgcccacctcggcctcccaaagtgctgggattacaggcgtgagccaccgcgcccggccaac

SEQ ID NO: 11280 - RNA, 4854 nt, Homo sapiens
  source 1..4854: mol_type = other RNA
ctgaatagctgggactacaggtgcccgccaccacacccagctaatttttttgtatttttagtagagacggggtttcaccatgttggccaggatggtctcgatctcctgacctcatgatccacccacctctgcctcccaaagtgctgggattacagggttgagccactgcgcctagccttttatttatttatttatttttttgagacagtgtctcactgtttcccaggctggagtgcagtatcacaatctcggctcactgtgacctccacctcctggattcaagcaattcaggctggtcatgaactcccaacctcaggtgatccacctgccttggcctcccaaagtgctggtattacaggcataagccaccacacctggagttttagtcagagcttcagtgacctggaggaagggaaatatccaactccagccaactctatacatcctgacccaactaaagggtgggaaaaactgaagttcacagtgcagaagcacagactcactgcaagactgacatctaatccctggacaatagaatgctgcccctctccccacagcttatcatgattactagaggcctgcttacagcatttcctcttatccagtatgccatgtccagctaaggaaaaattacaagcatactaaaaggcaaaagttagtttaaagagaaagagtaagaaccagaaccagatatagcaggattgctgaaattatcagactgggaatttaaaacaattatgattgatatgccatgggttctactggataaagcagacagcatccaagaacagacaggcagtgtaaacacagagatggaaattctaagaaccacaaagaaatgctagaaattgaagacagtgtaacagaaatgaagaatgtctttggtaggcttattattggccaagaaacagccaactaaagagcttgagaatatatcagcagaaacatccacacctgaaaagcaaagagaagaataaaaaaacaagatataagaactgtgggataactacaaaagatgtatcctacatataaaggaaataccagatggaaagaaaaaaaaagggaaacaatgacagaatttctcaaaattaactcagacaccaaaacgcaaatccaggaggctaagcaaacaccaagaaggacgagcaccaaaaacctatacctaggcatatcatttaaaaataacagaatatcaaagataacaaaaaattttcatagaagccagagggggggaaatgctttaagtattgaggatcaagtataagaattacatccaactttgagcatagaaggaagaagtgaaggtaaaataaaaatgtttatttttctaatacttaattgatctgataacttctgaaaaatagctacaatgtattagattacatatgctaatttgtgtgtgtttataggcataaaagtgaaatatagtaatgatggaaggtctgagagggaggatttaggattattttgatagtataaggtactaacactactcaagaaacggtacagtattatcagaattcatgtacttattatggcatgtgaaatatttaaaggttataccatattccttaccttcccagggttctgaggtaattttacatgtgtaaaaaaaattctgtggaattaatgtaaggcttcctacatgcattacaggtaaaaggcttctctccagttcgacttcttacaccttctagaaggtagaaaacattaatgtaagcttttccacaatcctaatgggatttcagtccactccaagttccagtatggtgtatggggtcacattccttgcgttcacagtaaaagaaactttctttccttttttctcctctattttcacatggtctacgaccagacaacttgcatgtgaatattaaaatatagtgaacattcacaggctttttcatgctccttacattcatacaatttctctcctatgtgatttctcctgtatgtagaaaggactgaagactcaatgaaggctctcccacgtcttacattcatatagtttctctccagtgtggctttgcatgtgaatattaaggcttttggacaatctataaacgtttttgcttattgcttactgtattcacttgctagagccaccacaacaaaataccacagactgggtggctcaaacaagagaattttatttgttcaaagttctggaagcccaagatgaaggtgccagcagggttggtggctttgatagaaggatctgtcccagtgctctgtctttggcttgcagatggccatcatctgatgacttcacatcatcttctatttgttgtctcagttgtgtctttctcttcttatagggacaccaatcatattggattagggatgtactctaacagactcaatttaatcaaataattttcttttttttttttttttgagatggagtctcactccatcgcccaggctggagtgcagtggcatgatctctgctcactgcaacctctgcttcctgggttcaagtgattcacttgcctcagcctcccaagtagctgggattacaggtgcccaccacacctggctaaattttttgtattttcagtagagacaaggtttcaccatgttggccagggtggtctcaaactcctgacctcaagtgatccacccacctcagcctctcaaaatgctgggattacaggaattaagtaattttcatgcagcttcttctctccagagtgagttcattcatgtctttaaagtgaactggaacaaatgagagctttcccacatttattacatggacagtttctcactagtgaatttgttcatgtcttcgaagtgaacggggatgactgtaagctttcccgcattgctgacatttatagggtttctcttctgtgtgagttttttcatgaattctaaaggaactggaacacgtgaaggctttcccacactccttgcattcatagggtttctctccagtgtgagtcctttcatgtatttgaaatgaactggaatgactgaaggcctttccacattgtttacactcatagggtttttctccagtgtggattcgcatgtgaattttaaggtgggtggaatagttaaaagccttcccacattccttacaggtgtatggtttctgggcactgtgcgttcgcatgtgattattaagacatgagggatacccaaatactttcccacatatcttacactcacaggccttctcttcagtgtgagttctcaaatgtccactaagatttgaggaaactgcaaaggctttcccacattcaacacatacaaaaggcttctctccagtgtgagttcttatatgttgaataaggcgtgaggatgtaaggaaggatttcccacattccttacattcatagggcttgtctccactgtgagatcgtacatgcatactaaggcccgagtactgagtgaaggctttcccacattccttacatacatagggtttctctccagtgtgagttcttccatgtatctgaaatgagttggaataattgaaggctttcccacattccttacattcatatggtttctccccagtgtgggttcgcatgtgaatactgaggtaggctgggtatctatagccttttccacattccttacatttgtagggcttttttgcattgagggtttctataagcacagaaaggcttgtagagtcaataaaacctggcccataattcctccattcgtagagtttttctccattgtgagttctcatatgtgcctgaaggtatgactcattaatgaaggattttccacagtgactacattcaaatgacttttcttgtgtgctagttctctggtatacaatatttggtgtcaggctgaagattttttcactctgattaaactcagaaagtttctcaccagtagaggttttctcacacagggtaaggaaatcttttccatactgattacagtcatgagtgttccctgtactttgagttctcacgtgcgtcttaaggcatgagtgttcactgaagacttctccacattgctcacagtcacagagttcccttccattgtgttttccttccaattgtatcccaatggatgtctgacccctcaaaaagtcctgctgaagtatagaccactgggtttcaagtcgcatttcccatccttggagaactcctccctgaactgtccttgactcttcttgttccaaccaagagattagactgggtttgatgatctgacctcctactgtggccaggttcttgtagttctccagcatcacgtcactgtagaggcttctctgagttgagtccagtaaagtccactcctcctgggtgaagtccacagccacatcgtcaaaggtcactgaatccatgggacaaatcagcagctgccatcccgcgaggtgagaacgtgtcagaaccctcctttcattgatgtcaccatcacttcaggacacctcattaatctaaatggacagtggcaatctccattcctctttaaacagggttattgggattccggaacactcagaaatcgccaggtccctgaaccgggaagatcctggggacggagccaacgcggatgcaaaaggcagcaattattttcctgccggaaaaaaattcacaaacgctgctttggaggcctttggagaggggcgcacagatgaaaacaccctgcggacaccgtaactataaacccgactcctcccgaggagcgacggtccgagcggacgctagcgggcccagcagacacgagcagagcgggccaggcctctctaacgtccgggccaaacccgtccttcaccccaaaaccagttcatctcctcggaactcacccaggccagtgaggccttaactctgaaaggcaaaaagactctcaggcgctcacagccggcgtcacaaaagg

SEQ ID NO: 11281 - RNA, 4717 nt, Homo sapiens
  source 1..4717: mol_type = other RNA
ctgaatagctgggactacaggtgcccgccaccacacccagctaatttttttgtatttttagtagagacggggtttcaccatgttggccaggatggtctcgatctcctgacctcatgatccacccacctctgcctcccaaagtgctgggattacagggttgagccactgcgcctagccttttatttatttatttatttttttgagacagtgtctcactgtttcccaggctggagtgcagtatcacaatctcggctcactgtgacctccacctcctggattcaagcaattcaggctggtcatgaactcccaacctcaggtgatccacctgccttggcctcccaaagtgctggtattacaggcataagccaccacacctggagttttagtcagagcttcagtgacctggaggaagggaaatatccaactccagccaactctatacatcctgacccaactaaagggtgggaaaaactgaagttcacagtgcagaagcacagactcactgcaagactgacatctaatccctggacaatagaatgctgcccctctccccacagcttatcatgattactagaggcctgcttacagcatttcctcttatccagtatgccatgtccagctaaggaaaaattacaagcatactaaaaggcaaaagttagtttaaagagaaagagtaagaaccagaaccagatatagcaggattgctgaaattatcagactgggaatttaaaacaattatgattgatatgccatgggttctactggataaagcagacagcatccaagaacagacaggcagtgtaaacacagagatggaaattctaagaaccacaaagaaatgctagaaattgaagacagtgtaacagaaatgaagaatgtctttggtaggcttattattggccaagaaacagccaactaaagagcttgagaatatatcagcagaaacatccacacctgaaaagcaaagagaagaataaaaaaacaagatataagaactgtgggataactacaaaagatgtatcctacatataaaggaaataccagatggaaagaaaaaaaaagggaaacaatgacagaatttctcaaaattaactcagacaccaaaacgcaaatccaggaggctaagcaaacaccaagaaggacgagcaccaaaaacctatacctaggcatatcatttaaaaataacagaatatcaaagataacaaaaaattttcatagaagccagagggggggaaatgctttaagtattgaggatcaagtataagaattacatccaactttgagcatagaaggaagaagtgaaggtaaaataaaaatgtttatttttctaatacttaattgatctgataacttctgaaaaatagctacaatgtattagattacatatgctaatttgtgtgtgtttataggcataaaagtgaaatatagtaatgatggaaggtctgagagggaggatttaggattattttgatagtataaggtactaacactactcaagaaacggtacagtattatcagaattcatgtacttattatggcatgtgaaatatttaaaggttataccatattccttaccttcccagggttctgaggtaattttacatgtgtaaaaaaaattctgtggaattaatgtaaggcttcctacatgcattacaggtaaaaggcttctctccagttcgacttcttacaccttctagaaggtagaaaacattaatgtaagcttttccacaatcctaatgggatttcagtccactccaagttccagtatggtgtatggggtcacattccttgcgttcacagtaaaagaaactttctttccttttttctcctctattttcacatggtctacgaccagacaacttgcatgtgaatattaaaatatagtgaacattcacaggctttttcatgctccttacattcatacaatttctctcctatgtgatttctcctgtatgtagaaaggactgaagactcaatgaaggctctcccacgtcttacattcatatagtttctctccagtgtggctttgcatgtgaatattaaggcttttggacaatctataaacgtttttgcttattgcttactgtattcacttgctagagccaccacaacaaaataccacagactgggtggctcaaacaagagaattttatttgttcaaagttctggaagcccaagatgaaggtgccagcagggttggtggctttgatagaaggatctgtcccagtgctctgtctttggcttgcagatggccatcatctgatgacttcacatcatcttctatttgttgtctcagttgtgtctttctcttcttatagggacaccaatcatattggattagggatgtactctaacagactcaatttaatcaaataattttcttttttttttttttttgagatggagtctcactccatcgcccaggctggagtgcagtggcatgatctctgctcactgcaacctctgcttcctgggttcaagtgattcacttgcctcagcctcccaagtagctgggattacaggtgcccaccacacctggctaaattttttgtattttcagtagagacaaggtttcaccatgttggccagggtggtctcaaactcctgacctcaagtgatccacccacctcagcctctcaaaatgctgggattacaggaattaagtaattttcatgcagcttcttctctccagagtgagttcattcatgtctttaaagtgaactggaacaaatgagagctttcccacatttattacatggacagtttctcactagtgaatttgttcatgtcttcgaagtgaacggggatgactgtaagctttcccgcattgctgacatttatagggtttctcttctgtgtgagttttttcatgaattctaaaggaactggaacacgtgaaggctttcccacactccttgcattcatagggtttctctccagtgtgagtcctttcatgtatttgaaatgaactggaatgactgaaggcctttccacattgtttacactcatagggtttttctccagtgtggattcgcatgtgaattttaaggtgggtggaatagttaaaagccttcccacattccttacaggtgtatggtttctgggcactgtgcgttcgcatgtgattattaagacatgagggatacccaaatactttcccacatatcttacactcacaggccttctcttcagtgtgagttctcaaatgtccactaagatttgaggaaactgcaaaggctttcccacattcaacacatacaaaaggcttctctccagtgtgagttcttatatgttgaataaggcgtgaggatgtaaggaaggatttcccacattccttacattcatagggcttgtctccactgtgagatcgtacatgcatactaaggcccgagtactgagtgaaggctttcccacattccttacatacatagggtttctctccagtgtgagttcttccatgtatctgaaatgagttggaataattgaaggctttcccacattccttacattcatatggtttctccccagtgtgggttcgcatgtgaatactgaggtaggctgggtatctatagccttttccacattccttacatttgtagggcttttttgcattgagggtttctataagcacagaaaggcttgtagagtcaataaaacctggcccataattcctccattcgtagagtttttctccattgtgagttctcatatgtgcctgaaggtatgactcattaatgaaggattttccacagtgactacattcaaatgacttttcttgtgtgctagttctctggtatacaatatttggtgtcaggctgaagattttttcactctgattaaactcagaaagtttctcaccagtagaggttttctcacacagggtaaggaaatcttttccatactgattacagtcatgagtgttccctgtactttgagttctcacgtgcgtcttaaggcatgagtgttcactgaagacttctccacattgctcacagtcacagagttcccttccattgtgttttccttccaattgtatcccaatggatgtctgacccctcaaaaagtcctgctgaagtatagaccactgggtttcaagtcgcatttcccatccttggagaactcctccctgaactgtccttgactcttcttgttccaaccaagagattagactgggtttgatgatctgacctcctactgtggccaggttcttgtagttctccagcatcacgtcactgtagaggcttctctgagttgagtccagtaaagtccactcctcctgggtgaagtccacagccacatcgtcaaaggtcactgaatcctgataacaatctgttaggcagtcagccactattcttcctgctggtgtcttttcttcatgaaggcaaactgggtccccagaaagataatgtccatgggacaaatcagcagctgccatcccgcgaggtgagaacgtgtcagaaccctcctttcattgatgtcaccatcacttcaggacacctcattaatctaaatggacagtggcaatctccattcctctttaaacagggttattgggattccggaacactcagaaatcgccaggtccctgaaccgggaagatcctggggacggagccaacgcggatgcaaaaggcagcaattattttcccaggccagtgaggccttaactctgaaaggcaaaaagactctcaggcgctcacagccggcgtcacaaaagg

SEQ ID NO: 11282 - RNA, 4590 nt, Homo sapiens
  source 1..4590: mol_type = other RNA
ctgaatagctgggactacaggtgcccgccaccacacccagctaatttttttgtatttttagtagagacggggtttcaccatgttggccaggatggtctcgatctcctgacctcatgatccacccacctctgcctcccaaagtgctgggattacagggttgagccactgcgcctagccttttatttatttatttatttttttgagacagtgtctcactgtttcccaggctggagtgcagtatcacaatctcggctcactgtgacctccacctcctggattcaagcaattcaggctggtcatgaactcccaacctcaggtgatccacctgccttggcctcccaaagtgctggtattacaggcataagccaccacacctggagttttagtcagagcttcagtgacctggaggaagggaaatatccaactccagccaactctatacatcctgacccaactaaagggtgggaaaaactgaagttcacagtgcagaagcacagactcactgcaagactgacatctaatccctggacaatagaatgctgcccctctccccacagcttatcatgattactagaggcctgcttacagcatttcctcttatccagtatgccatgtccagctaaggaaaaattacaagcatactaaaaggcaaaagttagtttaaagagaaagagtaagaaccagaaccagatatagcaggattgctgaaattatcagactgggaatttaaaacaattatgattgatatgccatgggttctactggataaagcagacagcatccaagaacagacaggcagtgtaaacacagagatggaaattctaagaaccacaaagaaatgctagaaattgaagacagtgtaacagaaatgaagaatgtctttggtaggcttattattggccaagaaacagccaactaaagagcttgagaatatatcagcagaaacatccacacctgaaaagcaaagagaagaataaaaaaacaagatataagaactgtgggataactacaaaagatgtatcctacatataaaggaaataccagatggaaagaaaaaaaaagggaaacaatgacagaatttctcaaaattaactcagacaccaaaacgcaaatccaggaggctaagcaaacaccaagaaggacgagcaccaaaaacctatacctaggcatatcatttaaaaataacagaatatcaaagataacaaaaaattttcatagaagccagagggggggaaatgctttaagtattgaggatcaagtataagaattacatccaactttgagcatagaaggaagaagtgaaggtaaaataaaaatgtttatttttctaatacttaattgatctgataacttctgaaaaatagctacaatgtattagattacatatgctaatttgtgtgtgtttataggcataaaagtgaaatatagtaatgatggaaggtctgagagggaggatttaggattattttgatagtataaggtactaacactactcaagaaacggtacagtattatcagaattcatgtacttattatggcatgtgaaatatttaaaggttataccatattccttaccttcccagggttctgaggtaattttacatgtgtaaaaaaaattctgtggaattaatgtaaggcttcctacatgcattacaggtaaaaggcttctctccagttcgacttcttacaccttctagaaggtagaaaacattaatgtaagcttttccacaatcctaatgggatttcagtccactccaagttccagtatggtgtatggggtcacattccttgcgttcacagtaaaagaaactttctttccttttttctcctctattttcacatggtctacgaccagacaacttgcatgtgaatattaaaatatagtgaacattcacaggctttttcatgctccttacattcatacaatttctctcctatgtgatttctcctgtatgtagaaaggactgaagactcaatgaaggctctcccacgtcttacattcatatagtttctctccagtgtggctttgcatgtgaatattaaggcttttggacaatctataaacgtttttgcttattgcttactgtattcacttgctagagccaccacaacaaaataccacagactgggtggctcaaacaagagaattttatttgttcaaagttctggaagcccaagatgaaggtgccagcagggttggtggctttgatagaaggatctgtcccagtgctctgtctttggcttgcagatggccatcatctgatgacttcacatcatcttctatttgttgtctcagttgtgtctttctcttcttatagggacaccaatcatattggattagggatgtactctaacagactcaatttaatcaaataattttcttttttttttttttttgagatggagtctcactccatcgcccaggctggagtgcagtggcatgatctctgctcactgcaacctctgcttcctgggttcaagtgattcacttgcctcagcctcccaagtagctgggattacaggtgcccaccacacctggctaaattttttgtattttcagtagagacaaggtttcaccatgttggccagggtggtctcaaactcctgacctcaagtgatccacccacctcagcctctcaaaatgctgggattacaggaattaagtaattttcatgcagcttcttctctccagagtgagttcattcatgtctttaaagtgaactggaacaaatgagagctttcccacatttattacatggacagtttctcactagtgaatttgttcatgtcttcgaagtgaacggggatgactgtaagctttcccgcattgctgacatttatagggtttctcttctgtgtgagttttttcatgaattctaaaggaactggaacacgtgaaggctttcccacactccttgcattcatagggtttctctccagtgtgagtcctttcatgtatttgaaatgaactggaatgactgaaggcctttccacattgtttacactcatagggtttttctccagtgtggattcgcatgtgaattttaaggtgggtggaatagttaaaagccttcccacattccttacaggtgtatggtttctgggcactgtgcgttcgcatgtgattattaagacatgagggatacccaaatactttcccacatatcttacactcacaggccttctcttcagtgtgagttctcaaatgtccactaagatttgaggaaactgcaaaggctttcccacattcaacacatacaaaaggcttctctccagtgtgagttcttatatgttgaataaggcgtgaggatgtaaggaaggatttcccacattccttacattcatagggcttgtctccactgtgagatcgtacatgcatactaaggcccgagtactgagtgaaggctttcccacattccttacatacatagggtttctctccagtgtgagttcttccatgtatctgaaatgagttggaataattgaaggctttcccacattccttacattcatatggtttctccccagtgtgggttcgcatgtgaatactgaggtaggctgggtatctatagccttttccacattccttacatttgtagggcttttttgcattgagggtttctataagcacagaaaggcttgtagagtcaataaaacctggcccataattcctccattcgtagagtttttctccattgtgagttctcatatgtgcctgaaggtatgactcattaatgaaggattttccacagtgactacattcaaatgacttttcttgtgtgctagttctctggtatacaatatttggtgtcaggctgaagattttttcactctgattaaactcagaaagtttctcaccagtagaggttttctcacacagggtaaggaaatcttttccatactgattacagtcatgagtgttccctgtactttgagttctcacgtgcgtcttaaggcatgagtgttcactgaagacttctccacattgctcacagtcacagagttcccttccattgtgttttccttccaattgtatcccaatggatgtctgacccctcaaaaagtcctgctgaagtatagaccactgggtttcaagtcgcatttcccatccttggagaactcctccctgaactgtccttgactcttcttgttccaaccaagagattagactgggtttgatgatctgacctcctgataacaatctgttaggcagtcagccactattcttcctgctggtgtcttttcttcatgaaggcaaactgggtccccagaaagataatgtccatgggacaaatcagcagctgccatcccgcgaggtgagaacgtgtcagaaccctcctttcattgatgtcaccatcacttcaggacacctcattaatctaaatggacagtggcaatctccattcctctttaaacagggttattgggattccggaacactcagaaatcgccaggtccctgaaccgggaagatcctggggacggagccaacgcggatgcaaaaggcagcaattattttcccaggccagtgaggccttaactctgaaaggcaaaaagactctcaggcgctcacagccggcgtcacaaaagg

SEQ ID NO: 11283 - RNA, 4634 nt, Homo sapiens
  source 1..4634: mol_type = other RNA
ctgaatagctgggactacaggtgcccgccaccacacccagctaatttttttgtatttttagtagagacggggtttcaccatgttggccaggatggtctcgatctcctgacctcatgatccacccacctctgcctcccaaagtgctgggattacagggttgagccactgcgcctagccttttatttatttatttatttttttgagacagtgtctcactgtttcccaggctggagtgcagtatcacaatctcggctcactgtgacctccacctcctggattcaagcaattcaggctggtcatgaactcccaacctcaggtgatccacctgccttggcctcccaaagtgctggtattacaggcataagccaccacacctggagttttagtcagagcttcagtgacctggaggaagggaaatatccaactccagccaactctatacatcctgacccaactaaagggtgggaaaaactgaagttcacagtgcagaagcacagactcactgcaagactgacatctaatccctggacaatagaatgctgcccctctccccacagcttatcatgattactagaggcctgcttacagcatttcctcttatccagtatgccatgtccagctaaggaaaaattacaagcatactaaaaggcaaaagttagtttaaagagaaagagtaagaaccagaaccagatatagcaggattgctgaaattatcagactgggaatttaaaacaattatgattgatatgccatgggttctactggataaagcagacagcatccaagaacagacaggcagtgtaaacacagagatggaaattctaagaaccacaaagaaatgctagaaattgaagacagtgtaacagaaatgaagaatgtctttggtaggcttattattggccaagaaacagccaactaaagagcttgagaatatatcagcagaaacatccacacctgaaaagcaaagagaagaataaaaaaacaagatataagaactgtgggataactacaaaagatgtatcctacatataaaggaaataccagatggaaagaaaaaaaaagggaaacaatgacagaatttctcaaaattaactcagacaccaaaacgcaaatccaggaggctaagcaaacaccaagaaggacgagcaccaaaaacctatacctaggcatatcatttaaaaataacagaatatcaaagataacaaaaaattttcatagaagccagagggggggaaatgctttaagtattgaggatcaagtataagaattacatccaactttgagcatagaaggaagaagtgaaggtaaaataaaaatgtttatttttctaatacttaattgatctgataacttctgaaaaatagctacaatgtattagattacatatgctaatttgtgtgtgtttataggcataaaagtgaaatatagtaatgatggaaggtctgagagggaggatttaggattattttgatagtataaggtactaacactactcaagaaacggtacagtattatcagaattcatgtacttattatggcatgtgaaatatttaaaggttataccatattccttaccttcccagggttctgaggtaattttacatgtgtaaaaaaaattctgtggaattaatgtaaggcttcctacatgcattacaggtaaaaggcttctctccagttcgacttcttacaccttctagaaggtagaaaacattaatgtaagcttttccacaatcctaatgggatttcagtccactccaagttccagtatggtgtatggggtcacattccttgcgttcacagtaaaagaaactttctttccttttttctcctctattttcacatggtctacgaccagacaacttgcatgtgaatattaaaatatagtgaacattcacaggctttttcatgctccttacattcatacaatttctctcctatgtgatttctcctgtatgtagaaaggactgaagactcaatgaaggctctcccacgtcttacattcatatagtttctctccagtgtggctttgcatgtgaatattaaggcttttggacaatctataaacgtttttgcttattgcttactgtattcacttgctagagccaccacaacaaaataccacagactgggtggctcaaacaagagaattttatttgttcaaagttctggaagcccaagatgaaggtgccagcagggttggtggctttgatagaaggatctgtcccagtgctctgtctttggcttgcagatggccatcatctgatgacttcacatcatcttctatttgttgtctcagttgtgtctttctcttcttatagggacaccaatcatattggattagggatgtactctaacagactcaatttaatcaaataattttcttttttttttttttttgagatggagtctcactccatcgcccaggctggagtgcagtggcatgatctctgctcactgcaacctctgcttcctgggttcaagtgattcacttgcctcagcctcccaagtagctgggattacaggtgcccaccacacctggctaaattttttgtattttcagtagagacaaggtttcaccatgttggccagggtggtctcaaactcctgacctcaagtgatccacccacctcagcctctcaaaatgctgggattacaggaattaagtaattttcatgcagcttcttctctccagagtgagttcattcatgtctttaaagtgaactggaacaaatgagagctttcccacatttattacatggacagtttctcactagtgaatttgttcatgtcttcgaagtgaacggggatgactgtaagctttcccgcattgctgacatttatagggtttctcttctgtgtgagttttttcatgaattctaaaggaactggaacacgtgaaggctttcccacactccttgcattcatagggtttctctccagtgtgagtcctttcatgtatttgaaatgaactggaatgactgaaggcctttccacattgtttacactcatagggtttttctccagtgtggattcgcatgtgaattttaaggtgggtggaatagttaaaagccttcccacattccttacaggtgtatggtttctgggcactgtgcgttcgcatgtgattattaagacatgagggatacccaaatactttcccacatatcttacactcacaggccttctcttcagtgtgagttctcaaatgtccactaagatttgaggaaactgcaaaggctttcccacattcaacacatacaaaaggcttctctccagtgtgagttcttatatgttgaataaggcgtgaggatgtaaggaaggatttcccacattccttacattcatagggcttgtctccactgtgagatcgtacatgcatactaaggcccgagtactgagtgaaggctttcccacattccttacatacatagggtttctctccagtgtgagttcttccatgtatctgaaatgagttggaataattgaaggctttcccacattccttacattcatatggtttctccccagtgtgggttcgcatgtgaatactgaggtaggctgggtatctatagccttttccacattccttacatttgtagggcttttttgcattgagggtttctataagcacagaaaggcttgtagagtcaataaaacctggcccataattcctccattcgtagagtttttctccattgtgagttctcatatgtgcctgaaggtatgactcattaatgaaggattttccacagtgactacattcaaatgacttttcttgtgtgctagttctctggtatacaatatttggtgtcaggctgaagattttttcactctgattaaactcagaaagtttctcaccagtagaggttttctcacacagggtaaggaaatcttttccatactgattacagtcatgagtgttccctgtactttgagttctcacgtgcgtcttaaggcatgagtgttcactgaagacttctccacattgctcacagtcacagagttcccttccattgtgttttccttccttggagaactcctccctgaactgtccttgactcttcttgttccaaccaagagattagactgggtttgatgatctgacctcctactgtggccaggttcttgtagttctccagcatcacgtcactgtagaggcttctctgagttgagtccagtaaagtccactcctcctgggtgaagtccacagccacatcgtcaaaggtcactgaatcctgataacaatctgttaggcagtcagccactattcttcctgctggtgtcttttcttcatgaaggcaaactgggtccccagaaagataatgtccatgggacaaatcagcagctgccatcccgcgaggtgagaacgtgtcagaaccctcctttcattgatgtcaccatcacttcaggacacctcattaatctaaatggacagtggcaatctccattcctctttaaacagggttattgggattccggaacactcagaaatcgccaggtccctgaaccgggaagatcctggggacggagccaacgcggatgcaaaaggcagcaattattttcccaggccagtgaggccttaactctgaaaggcaaaaagactctcaggcgctcacagccggcgtcacaaaagg

SEQ ID NO: 11284 - RNA, 9840 nt, Homo sapiens
  source 1..9840: mol_type = other RNA
ctgaatagctgggactacaggtgcccgccaccacacccggctaatttttgtatttttagtagagacggggtttcaccatgttggccaggctggtctcgaactcctgacatcaggtgatccccgcctcggcctcccaaagtgctgagactacaggtgtgagccacgtgcccagctaggtggtgtgtaaactttaaaaaagcagagatttcatcccacaaatgcagactgggatctccacatgaccaggtgctgtggactgaactgtaaatgtcctccaaattcatatgttgaagccctaacccccaatgtggctcttcttggacatatggcttttaggaagtaattaaggttagatgaggtcataatccagcaagattggtggccttacaagagccatgtgcaggcaccaagaaaagcctacgtgaataagacagcaagagggtgctcaccatgttggcatcctccggcctcagatctgtgggggactgcgggggtgatgggacagggagagaacaaggagtggattttcttgtcctttctaaggaaggggctgggagggcgagggctgcactgggtgctgggaccaagggtccaggggcttggatctcttgtttacaaacccctacttctttcctgctatctagcccacacccctgatgctccccggaaaggagagcaaggatccttgaacacgcgttagcactagaaggaaactggagctcaccccagttgagccctccatttgacagacagggaagctgaggcccagggaggtgaggggacttgctcagtctttccaattgagtatgtggggcagaaggagtccccagagccccggccccagccaccatcctatttgactttccccaacaggcattctacctcagctaaagatgctgcctgcctctcacaggccctgaggagaagatggccacatcacaggatcgaacactaccacaaaactcctaggaagggacaggaaggtgagaatcctttcttttttttttgagacggagtctcgctctgtcgcccaggctggagcgcagtggcgcgatctcacctcactgcaacctctgcctcccgggttcaagtaattctcctgtctcagcctcccaagtagctgggactacaggtacccaccaccacgcccagctaatttttgtatttctagtagagacggggttccaacatgttggccaggctgctcttgaactcctgacctcaggtgatccacccgcctcggcctcccaaagtgctgggattacaggcgtgagccaccaagcccggcctgagaattctcttctgtcaatggtgtgggcctctcgacctcactaacctatattggcccagaggtgatggtgacaatttgagataacacaaagtctcaactatttacgaacctggtcatccagagagggccccggaattgctcaaatgaacagtaagaatcctgaggcagggtactgaccttggtaggtgaaataccgcctatactctcaagttttatggatagtgcagccaaattccactcggatgcctcacaactacttaaaattggctttttgaagcagcatttccctaactactcccaggaacaaagttctgtgaaatgttcatagagcttcattgaaaaaaaaaaaaaaaaaaaagctacaatatttttcttctaagatttattttataaacatgtaagaaaagttgtagatatttattgtgggtctggttatgcaagaacaatcttcctggacacagtgtgcgattctcagtatcaaaagcattctcttctttcagttcgtaaaagaaaaacatggtttaacttctaatttactgcttattataaggtttaaaagcaattactgtacttatgtatcgaacttatttgtgtagcaactaattcatctgtgaagccatggtttgctgtggcttcacagtaaattttgacttaagtctaaagcgtgtgttagcatctcaccgtaacttaatgcttcgagtgagaagtttgaggaatgctgctttaggcaaaagagccactggaggaatgagctctgctcttttcacctgctctggactgctctcactttcctcaccgacaggaccacaggcttaagaactggctcagcagtccttctttagggtctagcgcctgcctaccagcttcctctacttctatcccgggacagatgaatgcttttctaaaaaatattttggaccatctgcatgattccctagcaaatgctttagagagctggtaagcttcagctccgacatggccagatcatcaaaatttgaagtttactcaggtctatttaatgagatttttttttcttatacaaccatatgcacttctgaataatcttccctttttcgaatctggggctttcatctggaattagactaacctgcagacagtgatgccagaactgggctgggttaccataattcattcatttaccaaacactttcgaagcactacttactctgggctggcctgatgaaaggatacagagataacaccacaaagaaacttgctcattaggagcttgcttactggctagaaaggaaaatacaacatgaaaataaagcattgtacgtacatggcagaaaaatgactagcctgccagagggccccagagcctcagaggatggagccactcctgaggctggagggtttacaaactcatcccatctttacagaagacctgctagatgccaggcatgctggcaggcacaggggaaagcccactcaacaagcagacacggtccctgctctcacggagcttacagtctagcaagacaaactaggaacaagaaattacagtccagtgtagaggtgtgcagggttgtggggtacagtgatttggcattatacacacatttcgcttaaacacaatggtatttgtctgaaaaagatttaaaaaaagaaaaacaaatcagttgtttgggccattccgctggcccctccttcactccatgagcatagacaagagggcgggcccgggcaagctcatgcctctgctgcacctgcggcctgcctcagttcccaagctccccaaaagtgatcttctcgcctaaatgtggttctaacaccccaaaacaagtgatttttgcacaacacagccctaactgcaggccaatcacttcacctggtactcaaccaaacagtaatgtgttcccacatgggcaagaaatgactacatgggacctcaagatgttggtcttcaatagggcaccttccttagatttctaagaggaattttaattacactccatttttatcttaggcactgaccttagaactgaatcctggagagagctgagactcttctgtggcagtaccatgggacacatagaagtagcctataccctggctctggaagttggggactgcctcctagaagggcccctaagaccttaagttggtgaggggaagattgaggcgggagggggagaagcctgggcggaagcatgtcactggaggtagaaacagctctgtgcacagtctgtagggctagtgagatcaagatacatttagggaactggtgagcagagggcaggggagatggggagaacaggccagggatactgccagaggatagaccttggtgagcctcataacatgctatcaaaaagggtggaatttatgtatgtatgtattttttgagacaggtcttgctctgctgcccaggctggagtgcagtggcttgatcatagctcaccacagccttgaattactgggctcatgcgatcaggagtgtggaatttattctcggggcaatagtgaagctttggaaaacgttcaagcagaggaataacagaatcagatatatatttaagaaagttcatcctgaagcatgtgaaaaggtgcccgacatcattagtcattagggaaatacaaatcaaaaccacaatgagagccaggcgtggtggctcatgcctgtaatctcggcactttgggaggtcaaggcaggaggatcacttgaggccaggagtgctagacggcctgggcaacataacgaaaccccatctgtacaaaatgtattttaaaaagaaaaaataaaaacaaaaaactacaatgagataccacttcacaccagaaaataatgagtgttggtggagatgtggagaaactggaaccctcgcacactgctggtggaatggaaaatgatacagctgcttggaaaaaccacctggtggttcctgaaaaggttaaagataattatgactcagcaattccactcctaggtatatacccaagagtcatgaaaatacctgtccctgcaaaaacttgttcgggaatgttcgtagcaacactattcataatagccaaaaagtagggccaggtgcagtggctcacacctgtaatcccagaactttgggaggaagaggtgggcagatcacctgaggtcaggagttcgagaccagcctgaccaacatggtgaaaccctgtctctactaaaaatacaaaaaattagccagcgtggtggcacatgcctgtaatcccagctactctggaggctgaggcaggagaatcgcttgaaccccggaggtggaggttgcagtgggccgagatcgtgccattgcactccagcctgcacaacaagagcgaaactgtgtctcaaaaataaataatagaaatagaaatatatatatatagccctaaagtagaaacaactcaaatgcccattaaccaatgtggattaaaaaaaaggtggcatacccataaaatggactattatttggcaattttaaaaaatgaaatactgatagaagctatgacatggatgaacctcagaaatatgttaagaagccagtcacaaatagacacatagtatatgatcccatttatatgaactatccagaacaggcaaatccacagagagagaaggaagatcagtggtggccagaggctaagagggaagagggaatagggagaattgctaatggactcagggtttctttgggtgatcaaagtgttttaaaattgattacggtgctggtgcataactgtaaatatactaaaagccactcaagtgtacactttaaatggctgaactgtatgcaaattacatctaaattaagctggtaacaacaacaaaggttcatcccgctgcagtgtgcagaatggagacagggcagagaccagtgaagaggctgctgtacaaatgcagctggaaagggcagtggctgaagaacggagaggggttcacaggatcagactacaagggggccagaggaggagactacatcctgaggacgccacaaattatcctgggtacctggtaactctccagagaggagagtgggaaacaaatgaggtatctgcaattatcatcaagcagcaaacatgtatgtaaaatctcctacacataagactaagaggaacacacaaagtgtgcagccctgtgcccacatgtgtggggagtgtccagggtaaaatcacgcccagctgcctgccacgggcctgtcctgactatccattcttactcttaaactccaaagaaaaggcctcatcattcaggacacactcaagatgttgcaagatctgagtgactgagagtgggcaggagggttagagaaactaataaggccagtaactccgagaagtaaaaatctttaaagctgcctttctgggttctctctgtgtgtctgtgaaaactgtaaggttactcgagtgtgtatttctcttggttacatcaaagacccagttttgactgcacaccacctccttccagaatggcttcgctgatctgtagcaggagactgctgagtgctgaaaggccgtggaacaaatggacctgagctgctggtgtaaaaccaaaaggaaagtctgtgaaggagcatattctaaaccctgcagaggcatgccagctgggacgctgaccacaagacatctttgccccgtcagtagaagcagagactgtgctgggatgggaataagcccctgtctacacctcatgcgcgccctcagttgtctccctggcgcctcctccacctgcagtagaaattcatgctggcgagcccactgccgtcacagcttgggaagagtaaaccgccactgagatgcaccaacaaagccaggaattctggtaacagcccactcaactgctagacgggaaaactgaggcccaggtccatggagcagagccaggggttggcatccaggtgtccgattctcaggcccccgcactcctcactctaccaactccccaaaccctgacccttcctaagaacctggctctcagctgtatgcttcacagggaaagaaaagctgagaaatctcagatgtcttaagtctcaactggcagagaaaccagaaccatctctttcctagaatcctaataagaagctgaaatatatcatggttatatcctctaatctctctaaagggagggagaaaaagcaaggttaatcaacaaaatatgggacaatacagtttttgttgcagctctcaaatcttgcagccctttacttcctttattaataacagtgttctgcattaattcgtgccacagtgtaatcaactatcaatgtgaccattagctccgccacaagtaaagatcgacaggatccaggctgcactgtgtgcacaacagcccaggcaggtgaagagtcgtgacatcgcaaaaaggaccacggtttattaccatctctaacgcccatgttccagcaaaccgaagaaaaacactgtttcttaaaactgcagaggaatacaaaattaaatactacaaaacaaaaatcagacaggaagacgaaacaatctacctcctcctaatggtaaaataatctgaaaggagtttaaaaataaatgaactaaaatttttataactattatcttttctgccaattttgaagatgtcttcaggtgccacaacgtggggacagaaagaataaatatcaatgtataacttctagagtgataataaacaacaggaccccatctcagatggatggattttttttcctactggagccaaaaaacaagctgaactctatgtacaacagacagactatacaactaggagcatttaaaaataataagactcctctctctgccttcttccaaagaatagaatatatatttaacagcacaaaagacgacaccacttgagcttcccctttagccaacaggaagaatttccacatataaaaattaaaaatttaaactttcaaatcattcatgttttaaacataatacagacttaaaaattcttcaacattgacccataatcccaccccagcacaaaaatcaaccccaaatccagacgtcacagttttttgttcctaaaaatcccacagcactgaacttgatcttcacatcaagctgacagcacgtaagaggcccatgccatgagcaatccccgagggaagaacggaagcacagtcaatgctgcagctcttatctacctgggcggcactggtgcacctctgaggtcaggtccgtgagattcgccccacactagggtcccggaagggtgagctggccgcttccctcctcttccccctcgaaggatgtccaataagcacctgggaattgacttttcttgggaaaagggtgctggtaacagctgtcagggccaaggcaatagtgagaagttcagttctctgctctttggatgaactgtgtaaaacatttcttttaaaagacacaatgttaaaaatattaagaaaaatgtctacaaaatctggagggctgcctttttctcaaagggtaaagcctgtggggtggtgggaaaggaatcgagggcccagaactacaactctgcagcgaaagatagagatgcccttgaaaatgtgtcacattcttaagatgtcttgccgaagtagcaagagcggagggtgactgtgtgagcaggagcgagagggcgccagctcctgcgggggaggttcctactgcgcgccccaccctgtgcaagaatgtcaggctttagggcagctgccataggccccaggggcatcaggactctgcctctgaaccagagctgctttcccgactaacttcaatctggagagatggtaagttatctaaccggctcttcttttggcgagactgctctttctccttaatcagagccccccatgccctttgcagctcagagtcgtcttcctcagcgccaggcgccctgtgatccactttcttcgtattcttttctttggtcttgggtgcagatcctaggcgagtccataaattacctgatttcttctcccgagtatcggcgtagaggcctttactatcctgcctgggaacacctagcctactatgcacatcagaagagggctctctccgaacgacggggttactactaaaagccttttccggagaatgtggtctttttcctaaccgctggcgtatatctgatttagtactgctgactggtggccgtggacgggagtgctgacgtttctcatctaatagatgtcggacatctgcaaatttctcaggtggtaatttgttaccaattcggtttttgatattgcttgaagatacactatctgccctcatggagttcctaatatttttcaactgagattccacttcgtcagcatacatagtcattttcatgcttttctttggtgaaggcgtggaaatcattttcagttctagatcatagtccatttcatctgagtctgagctgctggcactggatcgtctagacgcgctccgctcccggggctgcttgagagccgggagctcctcgtggtactctaccaccactctgtcatctgcatccatgtcctggtcttcttcttcctcttcctcttcctcctcctcctcctcttcctcctcttcaatgggttcctcgggaacattcactagcccagaatgtcgatgtttatacgacgtcaagccaacgtcatccccaatcagggctctcttcttgatcacgtcccgctgaatacgacgggaatgatatcttcgcttccatgaattgctaagaattcctttcatgcctccataatttggattcccatatttcatgtaatactgacttcttctggctgctccaagttcctttttgtcatcttttgtagcaaatctcatgaataacctatttcctttagcaagtttgttagctggacgaagatcgtttcttaacaaagactcctcttctacctgagacaacgtatccaactctacatcacttgagttctcatcttcaacctctccttcttcagcttcatcatcatctgaactgtcttcctgcttgtcttttttccttttctcagctgacttgtcctcactggcatccctgcttctgatcttatcctgtgcaggcagggagctcatattgataagtgctcgtgtggctgtcatttcatccagccaaactacattacaggaggtatcatccaaccattcgatgtgagctggaggatattctttaaaataggaaaagacatcttgggtgctcatctcatctactccgcaaatatagattgtctccagtctcaccttggggattgctttcttcatcatgtctcggtccaaggctacatttctttgggcaagatttacttccgatcgaaaatggaagcgcttggctcgctgctctttcttttcaattgcttccttggaggtgacatcaattccagtgatgaagctgccagccttgttttcatatcttctgctcgtgtccgggatcagttccttgagcgagcgccgcacaggcacgatttccagctcgccctcctccacctccatgggctccggctcgccacggtcaacaccggactccgcctcaggggacgggagccccagggccggccccgccggggcctccgccttcaccgacacccgcaggccccgtacggccgccatcgctgcctgccggccgcaccact

SEQ ID NO: 11285 - RNA, 2257 nt, Homo sapiens
  source 1..2257: mol_type = other RNA
ctgaatagctgggactacaggtgcccgccaccacacccggctaattttttgtatttttagtagagacggggtttcaccatgttagccaggatggtctcgatctcctgacctcgtgatccacccgcctcggcctcccaaagtgctaggattacaggcgtgagccaccgcgcccggccatgaatatttattttcacacacaaaagtccctcagacattgattcttaaattcaaaacaccaaaggcattgtatatgccttttcatgttttctaattgtgaagaaaataaattttacttaaaatgctaatatttgaataaagtatgcattcataattatgttcttgtctttaaagttaatttttcaaacagaactaaatcagttttatcttcagtagatcttttagaaaggaagcaatcctacctcatctaattagagtttagtcctactaggaagatacactacaaatatttattgtggcaatctttgaaagcaaaatgaaaggtgattttggtttccttttctatatgttcttgtattacatttttcaggtttttctctaagttcttttctgtgatttttaaatcagggaggaaaaattcattcagtctaaacacttaatatttcttctacaagaagtatcctcatggctattttgttattttgtttcacttaggggaaaatggatttgttggcctcaaatagctgctttattagatgcaatgaagcaggggacatagaagcaaaaagtaaaacagcaggagaagaagaaatgatgaaggtaatgatgacattttatacagatgactgcattcacacatgcgatgtgactgtatctctttaaaatgttaagtcatcatttactgtcactttgaagatttacttaatagctttttataatgtggtgtttcaaatagactcatttttaattacaaatcgcatagttgatggcttgtttatacagtgtggtagagaaatcagtgcatctaggagctaccttgccattatctccatggattagtatcttttactggtagttccacatgctctttttatgctttcattttcttgttttcttgcttgtattttaaaatctaatttttaaaatagataacatgtacacgtggtccaacatttttaaataaaagcataagaagatgaagacatatgcctgccatgcatcttgctcacctatgtcccagctcctgttcctctttccctttgttttgtttttttatagcctcctaaaatttctttataaacatatgaatatatttataattttcaactgtcttacactaaaggcagcctcctctatagttttctcgactttgatttttttttctttaaaattgtatcttggagagttttctactattagtttgaatgtagaaagctttctctttttcttgcttctcctctctttctctctctctcttttttaacgccacataatattccattttagggatgtacctttatttatttagtcttttatagatggaaatttaggctgtttccagtcttttgctcttataaacagtgctgcagtacataacattgaatatgcatcaatttgtagatgtgcgggtggacctgaagataaatttcaagaagcagaattaccaggtcggggtacacgcatttgtatttatgtaatgcttgagcttctgtgatgataatcactctatgaaacataaaaaatcatagcagaacttctggggccttagcccttacattttaaaaatatttttagtaatagtacccgtcttctttgcattaggagaaacatgaatcacataaaacatgatttttattttatttttaaaatttgtgtgcgtcactaagctggaaataaaagttccttattccaggctaaattccctcatccgtagtcagacgcgttatccattgcaccagtggcctgtgccctccctaaccctactctttgttttacatcattgtaaaagttacacagacatcttcatatcaaggtgaaattctaaataatactgttaatataacctagataaatcaggtagttaactggaatttgatgaaaacatttaaggcttaattttttagactcacaaaagccactgatctttaatgataaacatatatcaggatgtgtctaaagaataactccccccttcttgacacatggcttttctgtgtcttggcattccatcgcagtactgagcatcctgaaccttgctttgtttgtctcttttgggaatcactggttgcatccagtctga

SEQ ID NO: 11286 - RNA, 4588 nt, Homo sapiens
  source 1..4588: mol_type = other RNA
ctgaatagctgggactacaggtgcccgccaccacacccggcttattttttgtatttttagtagaggtggggtttcactgttagccaggatggtctcgatctcttaacctcgtaatccacccgcctcggcctcccaaagtgctgggattacaggcgtgagccactgcgcctggccttgggttgttatactggggtcttgaataatcattaaaggtgaaatgaaaataatttccttttgaggtggtcaattttgtgagatggattcttgttaggcagctgtcatggaaagatgatttagttcagttgacattaataatacgcatggtaatcctaacaggtgaatgtggttcaaactaaattgccagggaattgtcatggtctagaaaagccactctctccagtagactgctcacacagctacatgtcagccctcctcactgtgaaagtgacagacaccctagcatttttattcatctcccttaggtgcctcaactttttctcccactctcagctgaaaagagctacatctaccatttcatctacttagtgtattttcttattggctatgttaaaaaattacaaacataacaattatgaatgaaaaataactccatggctgggtgcagtggctcacacctgtaatcccagcactttgggaggctgaggcgggtagaccacaaggtcaggagttcaagaccagcctggccaagatggtgaaaccgtctctactaaaaatacaaaaattagccgggtgcagtggcaggcacctgtaatcccagctgcttgggaggctgagggaggagaatcagttgaacccggagggtggagattgcagtgagactctcaaaaaaacaaaacaacacaaaaaaatctcctaagatgattaaaacaaacttgcttctacaataaaccgtaaactcaccgtatctagtgattctgtacattaaatcttttgaacatgtttaccaatttggtgttatgaaaaattttttagaggttgtgtatgggctgggcacaatgactcatgcctgtaatcccaccactttgggaggctgagacgggcggatcactcaaggacaggagttcgagatcagctggggcaacatggcaaaaccccatctctacaaaaagtacaaaaattagccaggcgtgcactaattagtgggctggaccattactggtgtgtgtatctctagtctcaactactcagaggctgagctggcgagatcagtggagcccaggagattgaggctgctgtgagctgtggtcatgccactgcactccagccgggatgacagagtgacaccgtgtctcaaaaaaacaaaaaacaaaaaattgtgtctgtactccactttccaactggatatagtgtccatatcaaggtcatctaaataaatataatgttttggagagagttgttttttttttttttttttttgtgacggagtctcgctatgttgccgaggctggagagcagtggcgcgatcttggctcactgcaacctctgcctcctgggttcaagtgattctcctccctcagcttcctgagtagctgggattacaggtacccgccaccaggcccagctaattttttgtgtttttagtagagtcggggtttcaccatgttggacaggctggtctcgaactcctgaccttgtgatttacctgccttggcctcccaaagtgctgggattacaggtgtgagccactccactcggcacttttttcttttttttgagatggagttttgctcttgttgcccaggctggagtgcaatggcacaatctcggcttactgcaacctccgcctcccaggttcaagcgattctcctgcctcagcttcccaggtagctgggattacaggcacgtgctaccacgcccagctaatttttgtatttttagtagagacggggtttcaccatgttggacaggctggtcttgaactcctgacctcaggatttccacccgtctcagactcccaaagtgttgggattacaggcgtaagccactgcacccggcctccaggctcaagcaattcttatgcctcagccacatgagtagctggtattacaggtgtgtgccaacatgcctggcgaatttttgtatttttagtagagatggggtttcgccatgttggccaggctgttcttgaactcctggcttccatcagttctcccatcttagcctcccaaagtgttgggattacaggtgtgacccactgcaactggccaggcacttcaatttttttttttttgctctgtcaccaggctggagtgcagtggtgcgatctcggctcactgcagtctccgcctcgcgggttcaggcaattctgcctcacccttctgagtagctgggactacaggcatgccccaccatgcccagctaatttttgtatttttagtagagacggggtttcaccatgttggccaggatggtctcgatctctggaccttgtgatccgcctgcctcggcctcccaaagtgctgggattacaggcgtgagccaccacgcccagccaggcacttcaaattttttgtctctgtgtgtctgcgaataactgagaaagtgccacagtattgatttgggggttacaaacatattttagtgagtaggcaaattctcaaatacaaaatctatgaataaggatcaagtatacgttcatttggcattttaagtaccccaggttccctcattatctgagggagggcagcatatgaaacttatttagacttcttcttaaacatttaatgtaatttaatttatttgagacaggatgtctgttgcccaggctggagtatagtggcgcgatctcggctcagtgcaatctctgcctcccaggctcaagcaattcttatgcctcagccacctgagtagctggtattacaggcgtgtgccaacacaccctgtgaatttttgtatttttagtagagatgggattttgccatgttggccaggctggtcttgaactcctggcctcaagtgatccgcctgccttagcatcccaaagtgctgggattacaagtgtgagccaccgctcctgggctagaactcttttttttttgagatggagtcttgctctgttgcccaagctggagtacagtggcgcaatcttggctcactgcaacctctgtctcccgggctcaaacaattcttatgcctcagcctcccaagtagctgggattacaggcacgcggcaccacacccagctgatttttctatttttagtagagatggggtttcaccacgttggtcaggatggtctcgatctcctgacctcatgatccgcccaccttggcctcccaaagtgctgggattacaagtgtgagccaccacgccccgcctagaactcttatagagaatgaagaatgcgttttgattttcttttttgcatatccaagacattgcactcaagtttctgaatcggcctattaggttggtgcaaaagtaatagtggcttttgccattaaaaattaaaaatggcaaaaaccacgattagttttgcaccaacctaacatttaggaaaatggagagttccacgaaggtgggaatttctgtctttttcatttatgctgtctatggtcagcagctagaacagcagtgcacacacagcaggtgctcagccagtcggtatttgttgggtgaatcaaggaatgaaaatcacattcaagccaatacacgtgattaaactactgttgtatcattgggctgcgacggttacaagtccacaaactgtttaactggacatatgtgaggtggtaaatccctccattttacaggtctttgggaagttctggggccaggaaatccaaatttgataataggattttctcaactgaactcagggcagagcacagatggtctgagtgaacgccctgtgtgacaggtgccttcctgcaggtaggaacacttcctctgcagtcagagggagaagaaaacatcaggagctggatgtgatttcagatctgcaccgagaaacatgctgatttcactggggatgtggcagtcccaggtgaaggctggctaggtcataattgacatctcctccctgtctctgctctcagacatggagttgattatgctttttaaatactttatgaattccatccggatctcctcagggtcatcttccaggtttgagtgcaccagcttcagcttgttcaagggtggcgacaaagacaggcttcctttatcatctccagagcctggtttgtggtgtgcaattagcatacactgtgtgtcctgtaaggacggctgttggacaaagcaggaataccacatctccatttccttccggtggcttgggatgtcagcattgaagacgatcaccactccatgagcatccttcatcagggccggccagcaggactcaaacctcactccttgggttgggctgtattcagtgatgtcagaagattctgtcagaaagttggccaaaacagtttttccactctcgcaaggccccacgaagaggatcttggctttcagcatagttgtccgccgcggcttagccggccggagcccacgggaggcggcgcgtcaggacggagctctacttggccgctttcgtttccatggcgacggagagaggccc

SEQ ID NO: 11287 - RNA, 4678 nt, Homo sapiens
  source 1..4678: mol_type = other RNA
ctgaatagctgggactacaggtgcccgccaccacacccggcttattttttgtatttttagtagaggtggggtttcactgttagccaggatggtctcgatctcttaacctcgtaatccacccgcctcggcctcccaaagtgctgggattacaggcgtgagccactgcgcctggccttgggttgttatactggggtcttgaataatcattaaaggtgaaatgaaaataatttccttttgaggtggtcaattttgtgagatggattcttgttaggcagctgtcatggaaagatgatttagttcagttgacattaataatacgcatggtaatcctaacaggtgaatgtggttcaaactaaattgccagggaattgtcatggtctagaaaagccactctctccagtagactgctcacacagctacatgtcagccctcctcactgtgaaagtgacagacaccctagcatttttattcatctcccttaggtgcctcaactttttctcccactctcagctgaaaagagctacatctaccatttcatctacttagtgtattttcttattggctatgttaaaaaattacaaacataacaattatgaatgaaaaataactccatggctgggtgcagtggctcacacctgtaatcccagcactttgggaggctgaggcgggtagaccacaaggtcaggagttcaagaccagcctggccaagatggtgaaaccgtctctactaaaaatacaaaaattagccgggtgcagtggcaggcacctgtaatcccagctgcttgggaggctgagggaggagaatcagttgaacccggagggtggagattgcagtgagactctcaaaaaaacaaaacaacacaaaaaaatctcctaagatgattaaaacaaacttgcttctacaataaaccgtaaactcaccgtatctagtgattctgtacattaaatcttttgaacatgtttaccaatttggtgttatgaaaaattttttagaggttgtgtatgggctgggcacaatgactcatgcctgtaatcccaccactttgggaggctgagacgggcggatcactcaaggacaggagttcgagatcagctggggcaacatggcaaaaccccatctctacaaaaagtacaaaaattagccaggcgtgcactaattagtgggctggaccattactggtgtgtgtatctctagtctcaactactcagaggctgagctggcgagatcagtggagcccaggagattgaggctgctgtgagctgtggtcatgccactgcactccagccgggatgacagagtgacaccgtgtctcaaaaaaacaaaaaacaaaaaattgtgtctgtactccactttccaactggatatagtgtccatatcaaggtcatctaaataaatataatgttttggagagagttgttttttttttttttttttttgtgacggagtctcgctatgttgccgaggctggagagcagtggcgcgatcttggctcactgcaacctctgcctcctgggttcaagtgattctcctccctcagcttcctgagtagctgggattacaggtacccgccaccaggcccagctaattttttgtgtttttagtagagtcggggtttcaccatgttggacaggctggtctcgaactcctgaccttgtgatttacctgccttggcctcccaaagtgctgggattacaggtgtgagccactccactcggcacttttttcttttttttgagatggagttttgctcttgttgcccaggctggagtgcaatggcacaatctcggcttactgcaacctccgcctcccaggttcaagcgattctcctgcctcagcttcccaggtagctgggattacaggcacgtgctaccacgcccagctaatttttgtatttttagtagagacggggtttcaccatgttggacaggctggtcttgaactcctgacctcaggatttccacccgtctcagactcccaaagtgttgggattacaggcgtaagccactgcacccggcctccaggctcaagcaattcttatgcctcagccacatgagtagctggtattacaggtgtgtgccaacatgcctggcgaatttttgtatttttagtagagatggggtttcgccatgttggccaggctgttcttgaactcctggcttccatcagttctcccatcttagcctcccaaagtgttgggattacaggtgtgacccactgcaactggccaggcacttcaatttttttttttttgctctgtcaccaggctggagtgcagtggtgcgatctcggctcactgcagtctccgcctcgcgggttcaggcaattctgcctcacccttctgagtagctgggactacaggcatgccccaccatgcccagctaatttttgtatttttagtagagacggggtttcaccatgttggccaggatggtctcgatctctggaccttgtgatccgcctgcctcggcctcccaaagtgctgggattacaggcgtgagccaccacgcccagccaggcacttcaaattttttgtctctgtgtgtctgcgaataactgagaaagtgccacagtattgatttgggggttacaaacatattttagtgagtaggcaaattctcaaatacaaaatctatgaataaggatcaagtatacgttcatttggcattttaagtaccccaggttccctcattatctgagggagggcagcatatgaaacttatttagacttcttcttaaacatttaatgtaatttaatttatttgagacaggatgtctgttgcccaggctggagtatagtggcgcgatctcggctcagtgcaatctctgcctcccaggctcaagcaattcttatgcctcagccacctgagtagctggtattacaggcgtgtgccaacacaccctgtgaatttttgtatttttagtagagatgggattttgccatgttggccaggctggtcttgaactcctggcctcaagtgatccgcctgccttagcatcccaaagtgctgggattacaagtgtgagccaccgctcctgggctagaactcttttttttttgagatggagtcttgctctgttgcccaagctggagtacagtggcgcaatcttggctcactgcaacctctgtctcccgggctcaaacaattcttatgcctcagcctcccaagtagctgggattacaggcacgcggcaccacacccagctgatttttctatttttagtagagatggggtttcaccacgttggtcaggatggtctcgatctcctgacctcatgatccgcccaccttggcctcccaaagtgctgggattacaagtgtgagccaccacgccccgcctagaactcttatagagaatgaagaatgcgttttgattttcttttttgcatatccaagacattgcactcaagtttctgaatcggcctattaggttggtgcaaaagtaatagtggcttttgccattaaaaattaaaaatggcaaaaaccacgattagttttgcaccaacctaacatttaggaaaatggagagttccacgaaggtgggaatttctgtctttttcatttatgctgtctatggtcagcagctagaacagcagtgcacacacagcaggtgctcagccagtcggtatttgttgggtgaatcaaggaatgaaaatcacattcaagccaatacacgtgattaaactactgttgtatcattgggctgcgacggttacaagtccacaaactgtttaactggacatatgtgaggtggtaaatccctccattttacaggtctttgggaagttctggggccaggaaatccaaatttgataataggattttctcaactgaactcagggcagagcacagatggtctgagtgaacgccctgtgtgacaggtgccttcctgcaggtaggaacacttcctctgcagtcagagggagaagaaaacatcaggagctggatgtgatttcagatctgcaccgagaaacatgctgatttcactggggatgtggcagtcccaggtgaaggctggctaggtcataattgacatctcctccctgtctctgctctcagacatggagttgattatgctttttaaatactttatgaattccatccggatctcctcagggtcatcttccaggtttgagtgcaccagcttcagcttgttcaagggtggcgacaaagacaggcttcctttatcatctccagagcctggtttgtggtgtgcaattagcatacactgtgtgtcctgtaaggacggctgttggacaaagcaggaataccacatctccatttccttccggtggcttgggatgtcagcattgaagacgatcaccactccatgagcatccttcatcagggccggccagcaggactcaaacttagcatcgccaccacagtcccatagctcgaattcacagcccgtgcctttgttgttgctggtaacatgcgggttctcaaattctaggatcctcactccttgggttgggctgtattcagtgatgtcagaagattctgtcagaaagttggccaaaacagtttttccactctcgcaaggccccacgaagaggatcttggctttcagcatagttgtccgccgcggcttagccggccggagcccacgggaggcggcgcgtcaggacggagctctacttggccgctttcgtttccatggcgacggagagaggccc

SEQ ID NO: 11288 - RNA, 4709 nt, Homo sapiens
  source 1..4709: mol_type = other RNA
ctgaatagctgggactacaggtgcccgccaccacacccggcttattttttgtatttttagtagaggtggggtttcactgttagccaggatggtctcgatctcttaacctcgtaatccacccgcctcggcctcccaaagtgctgggattacaggcgtgagccactgcgcctggccttgggttgttatactggggtcttgaataatcattaaaggtgaaatgaaaataatttccttttgaggtggtcaattttgtgagatggattcttgttaggcagctgtcatggaaagatgatttagttcagttgacattaataatacgcatggtaatcctaacaggtgaatgtggttcaaactaaattgccagggaattgtcatggtctagaaaagccactctctccagtagactgctcacacagctacatgtcagccctcctcactgtgaaagtgacagacaccctagcatttttattcatctcccttaggtgcctcaactttttctcccactctcagctgaaaagagctacatctaccatttcatctacttagtgtattttcttattggctatgttaaaaaattacaaacataacaattatgaatgaaaaataactccatggctgggtgcagtggctcacacctgtaatcccagcactttgggaggctgaggcgggtagaccacaaggtcaggagttcaagaccagcctggccaagatggtgaaaccgtctctactaaaaatacaaaaattagccgggtgcagtggcaggcacctgtaatcccagctgcttgggaggctgagggaggagaatcagttgaacccggagggtggagattgcagtgagactctcaaaaaaacaaaacaacacaaaaaaatctcctaagatgattaaaacaaacttgcttctacaataaaccgtaaactcaccgtatctagtgattctgtacattaaatcttttgaacatgtttaccaatttggtgttatgaaaaattttttagaggttgtgtatgggctgggcacaatgactcatgcctgtaatcccaccactttgggaggctgagacgggcggatcactcaaggacaggagttcgagatcagctggggcaacatggcaaaaccccatctctacaaaaagtacaaaaattagccaggcgtgcactaattagtgggctggaccattactggtgtgtgtatctctagtctcaactactcagaggctgagctggcgagatcagtggagcccaggagattgaggctgctgtgagctgtggtcatgccactgcactccagccgggatgacagagtgacaccgtgtctcaaaaaaacaaaaaacaaaaaattgtgtctgtactccactttccaactggatatagtgtccatatcaaggtcatctaaataaatataatgttttggagagagttgttttttttttttttttttttgtgacggagtctcgctatgttgccgaggctggagagcagtggcgcgatcttggctcactgcaacctctgcctcctgggttcaagtgattctcctccctcagcttcctgagtagctgggattacaggtacccgccaccaggcccagctaattttttgtgtttttagtagagtcggggtttcaccatgttggacaggctggtctcgaactcctgaccttgtgatttacctgccttggcctcccaaagtgctgggattacaggtgtgagccactccactcggcacttttttcttttttttgagatggagttttgctcttgttgcccaggctggagtgcaatggcacaatctcggcttactgcaacctccgcctcccaggttcaagcgattctcctgcctcagcttcccaggtagctgggattacaggcacgtgctaccacgcccagctaatttttgtatttttagtagagacggggtttcaccatgttggacaggctggtcttgaactcctgacctcaggatttccacccgtctcagactcccaaagtgttgggattacaggcgtaagccactgcacccggcctccaggctcaagcaattcttatgcctcagccacatgagtagctggtattacaggtgtgtgccaacatgcctggcgaatttttgtatttttagtagagatggggtttcgccatgttggccaggctgttcttgaactcctggcttccatcagttctcccatcttagcctcccaaagtgttgggattacaggtgtgacccactgcaactggccaggcacttcaatttttttttttttgctctgtcaccaggctggagtgcagtggtgcgatctcggctcactgcagtctccgcctcgcgggttcaggcaattctgcctcacccttctgagtagctgggactacaggcatgccccaccatgcccagctaatttttgtatttttagtagagacggggtttcaccatgttggccaggatggtctcgatctctggaccttgtgatccgcctgcctcggcctcccaaagtgctgggattacaggcgtgagccaccacgcccagccaggcacttcaaattttttgtctctgtgtgtctgcgaataactgagaaagtgccacagtattgatttgggggttacaaacatattttagtgagtaggcaaattctcaaatacaaaatctatgaataaggatcaagtatacgttcatttggcattttaagtaccccaggttccctcattatctgagggagggcagcatatgaaacttatttagacttcttcttaaacatttaatgtaatttaatttatttgagacaggatgtctgttgcccaggctggagtatagtggcgcgatctcggctcagtgcaatctctgcctcccaggctcaagcaattcttatgcctcagccacctgagtagctggtattacaggcgtgtgccaacacaccctgtgaatttttgtatttttagtagagatgggattttgccatgttggccaggctggtcttgaactcctggcctcaagtgatccgcctgccttagcatcccaaagtgctgggattacaagtgtgagccaccgctcctgggctagaactcttttttttttgagatggagtcttgctctgttgcccaagctggagtacagtggcgcaatcttggctcactgcaacctctgtctcccgggctcaaacaattcttatgcctcagcctcccaagtagctgggattacaggcacgcggcaccacacccagctgatttttctatttttagtagagatggggtttcaccacgttggtcaggatggtctcgatctcctgacctcatgatccgcccaccttggcctcccaaagtgctgggattacaagtgtgagccaccacgccccgcctagaactcttatagagaatgaagaatgcgttttgattttcttttttgcatatccaagacattgcactcaagtttctgaatcggcctattaggttggtgcaaaagtaatagtggcttttgccattaaaaattaaaaatggcaaaaaccacgattagttttgcaccaacctaacatttaggaaaatggagagttccacgaaggtgggaatttctgtctttttcatttatgctgtctatggtcagcagctagaacagcagtgcacacacagcaggtgctcagccagtcggtatttgttgggtgaatcaaggaatgaaaatcacattcaagccaatacacgtgattaaactactgttgtatcattgggctgcgacggttacaagtccacaaactgtttaactggacatatgtgaggtggtaaatccctccattttacaggtctttgggaagttctggggccaggaaatccaaatttgataataggattttctcaactgaactcagggcagagcacagatggtctgagtgaacgccctgtgtgacaggtgccttcctgcaggtaggaacacttcctctgcagtcagagggagaagaaaacatcaggagctggatgtgatttcagatctgcaccgagaaacatgctgatttcactggggatgtggcagtcccaggtgaaggctggctaggtcataattgacatctcctccctgtctctgctctcagacatggagttgattatgctttttaaatactttatgaattccatccggatctcctcagggtcatcttccaggtttgagtgcaccagcttcagcttgttcaagggtggcgacaaagacaggcttcctttatcatctccagagcctggtttgtggtgtgcaattagcatacactgtgtgtcctgtaaggacggctgttggacaaagcaggaataccacatctccatttccttccggtggcttgggatgtcagcattgaagacgatcaccactccatgagcatccttcatcagggccggccagcaggactcaaacttagcatcgccaccacagtcccatagctcgaattcacagcccgtgcctttgttgttgctggtaacatgcgggttctcaaattctaggatcctcactccttgggttgggctgtattcagtgatgtcagaagattctgtcagaaagttggccaaaacagtttttccactctgtgaaaatgagtgcaaataaaggtctttgctcgcaaggccccacgaagaggatcttggctttcagcatagttgtccgccgcggcttagccggccggagcccacgggaggcggcgcgtcaggacggagctctacttggccgctttcgtttccatggcgacggagagaggccc

SEQ ID NO: 11289 - RNA, 4751 nt, Homo sapiens
  source 1..4751: mol_type = other RNA
ctgaatagctgggactacaggtgcccgccaccacacccggcttattttttgtatttttagtagaggtggggtttcactgttagccaggatggtctcgatctcttaacctcgtaatccacccgcctcggcctcccaaagtgctgggattacaggcgtgagccactgcgcctggccttgggttgttatactggggtcttgaataatcattaaaggtgaaatgaaaataatttccttttgaggtggtcaattttgtgagatggattcttgttaggcagctgtcatggaaagatgatttagttcagttgacattaataatacgcatggtaatcctaacaggtgaatgtggttcaaactaaattgccagggaattgtcatggtctagaaaagccactctctccagtagactgctcacacagctacatgtcagccctcctcactgtgaaagtgacagacaccctagcatttttattcatctcccttaggtgcctcaactttttctcccactctcagctgaaaagagctacatctaccatttcatctacttagtgtattttcttattggctatgttaaaaaattacaaacataacaattatgaatgaaaaataactccatggctgggtgcagtggctcacacctgtaatcccagcactttgggaggctgaggcgggtagaccacaaggtcaggagttcaagaccagcctggccaagatggtgaaaccgtctctactaaaaatacaaaaattagccgggtgcagtggcaggcacctgtaatcccagctgcttgggaggctgagggaggagaatcagttgaacccggagggtggagattgcagtgagactctcaaaaaaacaaaacaacacaaaaaaatctcctaagatgattaaaacaaacttgcttctacaataaaccgtaaactcaccgtatctagtgattctgtacattaaatcttttgaacatgtttaccaatttggtgttatgaaaaattttttagaggttgtgtatgggctgggcacaatgactcatgcctgtaatcccaccactttgggaggctgagacgggcggatcactcaaggacaggagttcgagatcagctggggcaacatggcaaaaccccatctctacaaaaagtacaaaaattagccaggcgtgcactaattagtgggctggaccattactggtgtgtgtatctctagtctcaactactcagaggctgagctggcgagatcagtggagcccaggagattgaggctgctgtgagctgtggtcatgccactgcactccagccgggatgacagagtgacaccgtgtctcaaaaaaacaaaaaacaaaaaattgtgtctgtactccactttccaactggatatagtgtccatatcaaggtcatctaaataaatataatgttttggagagagttgttttttttttttttttttttgtgacggagtctcgctatgttgccgaggctggagagcagtggcgcgatcttggctcactgcaacctctgcctcctgggttcaagtgattctcctccctcagcttcctgagtagctgggattacaggtacccgccaccaggcccagctaattttttgtgtttttagtagagtcggggtttcaccatgttggacaggctggtctcgaactcctgaccttgtgatttacctgccttggcctcccaaagtgctgggattacaggtgtgagccactccactcggcacttttttcttttttttgagatggagttttgctcttgttgcccaggctggagtgcaatggcacaatctcggcttactgcaacctccgcctcccaggttcaagcgattctcctgcctcagcttcccaggtagctgggattacaggcacgtgctaccacgcccagctaatttttgtatttttagtagagacggggtttcaccatgttggacaggctggtcttgaactcctgacctcaggatttccacccgtctcagactcccaaagtgttgggattacaggcgtaagccactgcacccggcctccaggctcaagcaattcttatgcctcagccacatgagtagctggtattacaggtgtgtgccaacatgcctggcgaatttttgtatttttagtagagatggggtttcgccatgttggccaggctgttcttgaactcctggcttccatcagttctcccatcttagcctcccaaagtgttgggattacaggtgtgacccactgcaactggccaggcacttcaatttttttttttttgctctgtcaccaggctggagtgcagtggtgcgatctcggctcactgcagtctccgcctcgcgggttcaggcaattctgcctcacccttctgagtagctgggactacaggcatgccccaccatgcccagctaatttttgtatttttagtagagacggggtttcaccatgttggccaggatggtctcgatctctggaccttgtgatccgcctgcctcggcctcccaaagtgctgggattacaggcgtgagccaccacgcccagccaggcacttcaaattttttgtctctgtgtgtctgcgaataactgagaaagtgccacagtattgatttgggggttacaaacatattttagtgagtaggcaaattctcaaatacaaaatctatgaataaggatcaagtatacgttcatttggcattttaagtaccccaggttccctcattatctgagggagggcagcatatgaaacttatttagacttcttcttaaacatttaatgtaatttaatttatttgagacaggatgtctgttgcccaggctggagtatagtggcgcgatctcggctcagtgcaatctctgcctcccaggctcaagcaattcttatgcctcagccacctgagtagctggtattacaggcgtgtgccaacacaccctgtgaatttttgtatttttagtagagatgggattttgccatgttggccaggctggtcttgaactcctggcctcaagtgatccgcctgccttagcatcccaaagtgctgggattacaagtgtgagccaccgctcctgggctagaactcttttttttttgagatggagtcttgctctgttgcccaagctggagtacagtggcgcaatcttggctcactgcaacctctgtctcccgggctcaaacaattcttatgcctcagcctcccaagtagctgggattacaggcacgcggcaccacacccagctgatttttctatttttagtagagatggggtttcaccacgttggtcaggatggtctcgatctcctgacctcatgatccgcccaccttggcctcccaaagtgctgggattacaagtgtgagccaccacgccccgcctagaactcttatagagaatgaagaatgcgttttgattttcttttttgcatatccaagacattgcactcaagtttctgaatcggcctattaggttggtgcaaaagtaatagtggcttttgccattaaaaattaaaaatggcaaaaaccacgattagttttgcaccaacctaacatttaggaaaatggagagttccacgaaggtgggaatttctgtctttttcatttatgctgtctatggtcagcagctagaacagcagtgcacacacagcaggtgctcagccagtcggtatttgttgggtgaatcaaggaatgaaaatcacattcaagccaatacacgtgattaaactactgttgtatcattgggctgcgacggttacaagtccacaaactgtttaactggacatatgtgaggtggtaaatccctccattttacaggtctttgggaagttctggggccaggaaatccaaatttgataataggattttctcaactgaactcagggcagagcacagatggtctgagtgaacgccctgtgtgacaggtgccttcctgcaggtaggaacacttcctctgcagtcagagggagaagaaaacatcaggagctggatgtgatttcagatctgcaccgagaaacatgctgatttcactggggatgtggcagtcccaggtgaaggctggctaggtcataattgacatctcctccctgtctctgctctcagacatggagttgattatgctttttaaatactttatgaattccatccggatctcctcagggtcatcttccaggtttgagtgcaccagcttcagcttgttcaagggtggcgacaaagacaggcttcctttatcatctccagagcctggtttgtggtgtgcaattagcatacactgtgtgtcctgtaaggacggctgttggacaaagcaggaataccacatctccatttccttccggtggcttgggatgtcagcattgaagacgatcaccactccatgagcatccttcatcagggccggccagcaggactcaaacttagcatcgccaccacagtcccatagctcgaattcacagcccgtgcctttgttgttgctggtaacatgcgggttctcaaattctaggatcctcactccttgggttgggctgtattcagtgatgtcagaagattctgtcagaaagttggccaaaacagtttttccactcttgggccttcggggctcattaacaccgggctcgcctccactacctcctccgggcagtggttggaatcaaggtctcgcaaggccccacgaagaggatcttggctttcagcatagttgtccgccgcggcttagccggccggagcccacgggaggcggcgcgtcaggacggagctctacttggccgctttcgtttccatggcgacggagagaggccc

SEQ ID NO: 11290 - RNA, 4601 nt, Homo sapiens
  source 1..4601: mol_type = other RNA
ctgaatagctgggactacaggtgcccgccaccacacccggcttattttttgtatttttagtagaggtggggtttcactgttagccaggatggtctcgatctcttaacctcgtaatccacccgcctcggcctcccaaagtgctgggattacaggcgtgagccactgcgcctggccttgggttgttatactggggtcttgaataatcattaaaggtgaaatgaaaataatttccttttgaggtggtcaattttgtgagatggattcttgttaggcagctgtcatggaaagatgatttagttcagttgacattaataatacgcatggtaatcctaacaggtgaatgtggttcaaactaaattgccagggaattgtcatggtctagaaaagccactctctccagtagactgctcacacagctacatgtcagccctcctcactgtgaaagtgacagacaccctagcatttttattcatctcccttaggtgcctcaactttttctcccactctcagctgaaaagagctacatctaccatttcatctacttagtgtattttcttattggctatgttaaaaaattacaaacataacaattatgaatgaaaaataactccatggctgggtgcagtggctcacacctgtaatcccagcactttgggaggctgaggcgggtagaccacaaggtcaggagttcaagaccagcctggccaagatggtgaaaccgtctctactaaaaatacaaaaattagccgggtgcagtggcaggcacctgtaatcccagctgcttgggaggctgagggaggagaatcagttgaacccggagggtggagattgcagtgagactctcaaaaaaacaaaacaacacaaaaaaatctcctaagatgattaaaacaaacttgcttctacaataaaccgtaaactcaccgtatctagtgattctgtacattaaatcttttgaacatgtttaccaatttggtgttatgaaaaattttttagaggttgtgtatgggctgggcacaatgactcatgcctgtaatcccaccactttgggaggctgagacgggcggatcactcaaggacaggagttcgagatcagctggggcaacatggcaaaaccccatctctacaaaaagtacaaaaattagccaggcgtgcactaattagtgggctggaccattactggtgtgtgtatctctagtctcaactactcagaggctgagctggcgagatcagtggagcccaggagattgaggctgctgtgagctgtggtcatgccactgcactccagccgggatgacagagtgacaccgtgtctcaaaaaaacaaaaaacaaaaaattgtgtctgtactccactttccaactggatatagtgtccatatcaaggtcatctaaataaatataatgttttggagagagttgttttttttttttttttttttgtgacggagtctcgctatgttgccgaggctggagagcagtggcgcgatcttggctcactgcaacctctgcctcctgggttcaagtgattctcctccctcagcttcctgagtagctgggattacaggtacccgccaccaggcccagctaattttttgtgtttttagtagagtcggggtttcaccatgttggacaggctggtctcgaactcctgaccttgtgatttacctgccttggcctcccaaagtgctgggattacaggtgtgagccactccactcggcacttttttcttttttttgagatggagttttgctcttgttgcccaggctggagtgcaatggcacaatctcggcttactgcaacctccgcctcccaggttcaagcgattctcctgcctcagcttcccaggtagctgggattacaggcacgtgctaccacgcccagctaatttttgtatttttagtagagacggggtttcaccatgttggacaggctggtcttgaactcctgacctcaggatttccacccgtctcagactcccaaagtgttgggattacaggcgtaagccactgcacccggcctccaggctcaagcaattcttatgcctcagccacatgagtagctggtattacaggtgtgtgccaacatgcctggcgaatttttgtatttttagtagagatggggtttcgccatgttggccaggctgttcttgaactcctggcttccatcagttctcccatcttagcctcccaaagtgttgggattacaggtgtgacccactgcaactggccaggcacttcaatttttttttttttgctctgtcaccaggctggagtgcagtggtgcgatctcggctcactgcagtctccgcctcgcgggttcaggcaattctgcctcacccttctgagtagctgggactacaggcatgccccaccatgcccagctaatttttgtatttttagtagagacggggtttcaccatgttggccaggatggtctcgatctctggaccttgtgatccgcctgcctcggcctcccaaagtgctgggattacaggcgtgagccaccacgcccagccaggcacttcaaattttttgtctctgtgtgtctgcgaataactgagaaagtgccacagtattgatttgggggttacaaacatattttagtgagtaggcaaattctcaaatacaaaatctatgaataaggatcaagtatacgttcatttggcattttaagtaccccaggttccctcattatctgagggagggcagcatatgaaacttatttagacttcttcttaaacatttaatgtaatttaatttatttgagacaggatgtctgttgcccaggctggagtatagtggcgcgatctcggctcagtgcaatctctgcctcccaggctcaagcaattcttatgcctcagccacctgagtagctggtattacaggcgtgtgccaacacaccctgtgaatttttgtatttttagtagagatgggattttgccatgttggccaggctggtcttgaactcctggcctcaagtgatccgcctgccttagcatcccaaagtgctgggattacaagtgtgagccaccgctcctgggctagaactcttttttttttgagatggagtcttgctctgttgcccaagctggagtacagtggcgcaatcttggctcactgcaacctctgtctcccgggctcaaacaattcttatgcctcagcctcccaagtagctgggattacaggcacgcggcaccacacccagctgatttttctatttttagtagagatggggtttcaccacgttggtcaggatggtctcgatctcctgacctcatgatccgcccaccttggcctcccaaagtgctgggattacaagtgtgagccaccacgccccgcctagaactcttatagagaatgaagaatgcgttttgattttcttttttgcatatccaagacattgcactcaagtttctgaatcggcctattaggttggtgcaaaagtaatagtggcttttgccattaaaaattaaaaatggcaaaaaccacgattagttttgcaccaacctaacatttaggaaaatggagagttccacgaaggtgggaatttctgtctttttcatttatgctgtctatggtcagcagctagaacagcagtgcacacacagcaggtgctcagccagtcggtatttgttgggtgaatcaaggaatgaaaatcacattcaagccaatacacgtgattaaactactgttgtatcattgggctgcgacggttacaagtccacaaactgtttaactggacatatgtgaggtggtaaatccctccattttacaggtctttgggaagttctggggccaggaaatccaaatttgataataggattttctcaactgaactcagggcagagcacagatggtctgagtgaacgccctgtgtgacaggtgccttcctgcaggtaggaacacttcctctgcagtcagagggagaagaaaacatcaggagctggatgtgatttcagatctgcaccgagaaacatgctgatttcactggggatgtggcagtcccaggtgaaggctggctaggtcataattgacatctcctccctgtctctgctctcagacatggagttgattatgctttttaaatactttatgaattccatccggatctcctcagggtcatcttccaggtttgagtgcaccagcttcagcttgttcaagggtggcgacaaagacaggcttcctttatcatctccagagcctggtttgtggtgtgcaattagcatacactgtgtgtcctgtaaggacggctgttggacaaagcaggaataccacatctccatttccttccggtggcttgggatgtcagcattgaagacgatcaccactccatgagcatccttcatcagggccggccagcaggactcaaacttagcatcgccaccacagtcccatagctcgaattcacagcccgtgcctttgttgttgctggtaacatgcgggttctcaaattctaggatcctcgcaaggccccacgaagaggatcttggctttcagcatagttgtccgccgcggcttagccggccggagcccacgggaggcggcgcgtcaggacggagctctacttggccgctttcgtttccatggcgacggagagaggccc

SEQ ID NO: 11291 - RNA, 2032 nt, Homo sapiens
  source 1..2032: mol_type = other RNA
ctgaatagctgggactacaggtgcccgccaccacacctggctaatttttttgtttctttttttttttcagtagagatggggtttcaccgtgttagccaagatggtctcgatctgacctcgtgatccgcccgcctcggcctcccaaagtgctgggattacaggcgtgagccactgcgcccagccaaggtgggggaatttatttttttaaaaaagcaaaacaggtttatttggctcaaaattctggtggaaatttcaagattgggcagctgcacctggtgagggcctcatgctacttcaactcaaggcagcaagtagaaggggagaggcatgcacaaagagattacgtggccatatggcgagagaggaagcaagagacaaccgcaggaaggctgactctctaaccagctctcatgggaactcacccctccacaaaggacactaacctatccatgagggatccacccctattacccaaactcctcctactaggcaccacctcctaacactgcctcattgaggctcaaatttcaataccattttgggcaggggcagaccacatgcaaatcacagcatggggtaatagtgggggcaggttgacacagggctgctgcctacccagcaccagctgtctcttggccccttccagatcctggcaatctggctacaggcatgggcccagccttggacacagatgtggccacaggaagctgttagctctccagatctgatcagcctgggagagcggcacaacaaaggctcccaaaggagagtcgggatcctcagctagcctcagctctgctacccacccatatgtgcccagaacaggaaagatacgtgtttcttactcctccgggactcctaggtgaagctgagaccaggctcttcttgagtcctctcagctatggtgcaaccaccagcctagcaaggaatcagaaacatcttccggaagagtcagcaccatagagggtgctgaatgggcaatgaagcatcccggagatgaaacatctgggcagtgaggcatcccacaggtgttgggctatgcagtcactccctttctcagaccgaggcaagtacataagcactctgggcccctaatcaggggcctggggccaggtgggatgaaaacagcagtgtcctgccacctgaacaactgctactcacgcaggccccacctggcctctcagagggaggaacctgggactcctgaaccagattcagtttctccttcaacagccgggacttttcgctcctgactgcagaaaaacagcttcaatgtgaccatccttgatagtccgaggctgagtaaaatggcctgaggaggcaaaatctgaaaagctctattaggtggcaaactgctgtcactagaagagttgaggcccccttctcctcccctgcctgaccgccttcattcctgggaatggaacaggttcttggggcaagggtgaatcctcgagcaggtcccaggatcactatcctcacctccccgcggcactgaatggctatagctgtaaatgtgcgtccacggggtcactgtccagccaccaggaccaggtgcctggccatctggggaatcggaaaacgctcagcgggatgctctggccacctcccctgcccccagttaagatgtagagcgttcaacctaaaatgcctagaaacaaagcccaggcccgggaaggtcgaacgagtgcgacgccgctccctcaagctcttccctcggagccgtctcatttcccaaaactcccaaacacatcacagagagaggtgttgagccaggtggtcactcccttttccagaaccacagcaagaagttgagcctgctgggctcctaacgaaggccctggggcccggtgggatgaaaagccctattaggtagcaaacagctgtcactagaggggttgaggcccccttctcccctgcctgacgacgacggcggcaggaactcgaccggcgccggacagctcgcaacttgccttaccaagcgtaaatctcggttcctcccaactacccgcggccacggcctccgcagcagagc

SEQ ID NO: 11292 - RNA, 4545 nt, Homo sapiens
  source 1..4545: mol_type = other RNA
ctgaatagctgggactacaggtgcccgccaccacatccagctaattttttgtatttttagtacagacggggtttcactgtgttagccaggatggtctcaatctcctcacatcgtgatccgtcagcctcggcctcccaaagtgctgggattaaaggcgtgagccaccgcgccccaccctggagcattttaaaaaatatttaaatgcatgatacaaaggtggcatctcaatggtgattgggtaaagataatcatataaataattgtgctattataattatgatgaatggtattaagaaaaaatacagattggtgtgaaatgttttaaatacaatgcgggttcttgtttcattcattacaccaaatacattccaaatgcaacaaatgttttaaagtacggctaaaattgcatgagagctaggaaagaaatggataaatatttttaaatcttgggtggaaagtctttctgagcacatcatgaaattcagtaatcacaaacaaaagatcagtaacctggactaagtaacaatgaaaactttcccatggcaaaaacaagcaaaagtcttataaataaagttgcaagacaaagagcaaatatggagaaatatgtgcaatatagataacaagcagcttgtggcttccctaatataaaaagagttgtgtagttatttagaataaatcacccccttcccaaataaaaaagtataggtcttcagctgaggaaacgttttctcctgtctctactgaactactctcccatactctgaagttgaaggaaggaggtataaccaatggcagttgctattactcactcttaccaggagtaagggccagtgcccttcacacacacaccccccacacacaacacacacaaatgtacacacaaacatagacacaatgcactcagctctcacacacacaccacatacacaccacacacacacatacgcacacacatgtatatacaaacatgcacccaatgcactcaactcaaatacacacaacacatatacaacacatatcttgggcagtttattgtagggtcatacctgcctgcacggtatgatctgtacctgtaccccctctgcgtaccactcagctgtttctaagttttgcactctatctggatccagaaagatgccagtgaacgtggtcacaaaggggacatgttctgcctgctccccaaggtggaatcagtgcatagagtcccgtggctgcctattttctggttcgggtcatgagaaagtcacttcctccctttgcaaaagggtactgtttttgtgaaatgaagccagggtacgctgcgtgcatatctgaagtcagatccttctgaggttctgccgttagcttgtccatcttcattgtcaatggtatcgggaaattcccctcctttccccagctttgttgggtcttcaagggtgactgaaggagaggttcttatgagtcattgcattgaaggccaccagccagacaccactgtgagccataaactgtcatataaaagcttttccaaccaccaccacaacaacaaaatattctcagaacatagatatacacagaatacggtccctgtgtcaacagtcacttgtgtgggctcagtgctgacaacggtgctgtggctactccaggtatgctgcaatccctctttgaagattgccatcagggctggaaacacatatttttggtattctgagtccacaagtgtaatatttttacatcgtgtttgattttcggaaatggttaaaagtcattcgccacatacttcagtttataaaagaaatgtccaactggctggaaagagtggtggaagggcagaggggtgggaatggttaatgggtaccaaaaatttagaaagactgaataagacctagtatttgatagcacaacagggtgactatagtcaatcataattgaatcgtacattaaaaaataactaaaagagtataattggattgtttataatacaaagtataaatgcttgaggggatagataccccattctccatgttgtgattatcacacattgcacacctgtatcaaaacatctcatgcattccatgaatatgtacaccatgtacccacaaaagttacaattaaaaataaaaaaagaaatgtccaacaggctaagttttaatgatatatattttatatggatatataatgtttttaccctacatagacagagaaaactgtaaagtaataagactaattgatgttcttttgcagctcataaacactccgaaggcaattcccaaaggtaacttctgccattttgatagtgaaaattttggtcagctgtctgatgcccacccagctttctactccagtgttctcatgttcctcatttgttgcttcactttctcttacgtgccccactgcaatttcaggtctcgagtcagagaacagactatttcctcttccccttaattaacctccatccatttgcttgattgtttgtggctccttctataagggatgggtggaggtgccttacagtgaaaagacaggtatacatacacacacactgtatatatatagattggaaattcaaaggcatgacattcctgggaaccaaaaagcctgtccaaagattagctccatagctagctcaagggctttcaaatgccagaaaagagaactagggcagccagaagacttggccccacaattcaagtattaacactgagcaattctgtgttataatttgcagcagttagaggaaatcccaaagtccacgtttttgttatttcagtaaatttttttggatctcactctgtcacccaggcgggagtgcagtggtgtcaccacggctcactgcaacctcagactcctgggctcaagcgatcctcctgcctcagcctcctgagtagctgggactacaagtgcacgccaccatgcccggctaatttttaaaactttttttgcagacatggggtctcgctatgttgccagggctggtcttgaagacctcccaaagtttagtaatcttatatgaactgcttttacttttctgcattgtacccagaaggtgatgttttacttaatatttagtcagttattttaaccagaaacttttaatactaagcaagggggatttcttcctttctatcacaattatactacattccatgtggacaactgtatctctggcagttaattctagaggtggaaattagggaagggggtagtatggaagcatacagcatttacaaaactggcaaaaaataaaataagtcaaggggaggctcagattctttctttggacaaaggtgggctttgaggaaagatcctcactcatcagaggccgagccctacactaaccacagtaatttgtattgatacccaatttagttcaggagctataaaaatgtatgtttgcggccaggcgtggtggttcatgcctgtaataccagcactttgggaggccaaggcgggtggatcacgaggtcatgagatcgagaccatcctggctaacacggtgaaaccccatctctactaaaaatacaaaaaattagctgggcacggtggcggatacctgtagtcccagctactccagaggctgaggcaggagaatggcgtgaacccgggaggcggagcttgcagtgagtcgagatagcgccactacactcccgcctgggagaaagagtgagactccgtctcaaaaaaaaaaaaaagtatgtttgcattattgcacataaaaattaaaaattgagagctatttgtattcatctattgagagaaacggtctctgggggttaggatggggacctgtccccattatagacccgttctggtctataatttacctaagacgagagcagaaagggttttaaatgctgatcctaagttgtcgtcggagggcagtaccccagaggacaggggaatcattcctaacactggcaggggccagaggctgacagctggcattgaacacctgaatgtcaggatattactcgcctctctctaattcttcccaatagagcggatacactctggactccctggggtggagcagctacatgggcagtttgtacttgttcctcttgtctcttcatctgcccataagcccaaggcactcagagtcttccctcactgacacccagcaagccggtgaacacaccggcccactgcattgggaagccctttccttttgctaaggactgcattcgtctatgctgcatcttgaggctgtgcagtatcacctcccctcctccatggtttttcttctctaggcctagcaggcaagggagaaggagagatgccagaagcctctgtctttccttccccattcgtttcttactgagtcttggagttaaattgttagttagtgccgggcgtgtggctcacacctgtaatctcagcactttgggaggcaaaggtgggcgaatcaactgagatcaggagtttgaaaccaccctggccaacatggtgaaactccatctctactaaacatacaaaaattacctgggcgtggtgggggggccctgtggtcccagctacatgggaggctgaggcaggagaatcacttgaacccgggaggcagaggtt

SEQ ID NO: 11293 - RNA, 2839 nt, Homo sapiens
  source 1..2839: mol_type = other RNA
ctgaatagctgggactacaggtgcccgccaccacgcccagctaatctttatacttttaatagagacggggtttcaccgtgtcggcccggatggtctcgatctcttgacctcgtgacccgcccgcctcggcctcccaaagtgctgggatgacaggcgtgagccactgagcccggccttctcttgacgtttaaactatgaagtcagtccagagaaacgcaataaatgtcaacggtgaggatggtgttgaggcagaagtaggaccacactttttcctatcttattcagttgataacaatatgacctaggtagtaatttcctatgtgcctacttatacacgagtacaaaagagtaaaacagagagactgctaaattaaagggtacgtgaagttcttcatagtaactccgtaaactggaacactgtcaaaaagcagcagctagtgaattgtttccatgtatttttctattatccaataagtgaactatgctattcctttccagtctcccaagcacttcttgtccccatcaccacttcggtgctcgaagaaaaagtaacaaatcaaggaacacaactaaagaaacacacacacaaaccaaagacaactacagcgtctgcaaaagtttgctagaagactgaaactgttgagtataaggatctggtattctacgatcatgagttcacttcagagtttgttcaagacatacgtttcgtaaggaaacatcttagttagaagttattcagcagtaggtaccatccctaagtatttttcaccaaattcgtgacaataaagagctatctaaccagaaaaattagcgagtaccggcaccatccatagggctttgtctttacgcttcattagcacttaccatgccttacaatgtctaggattgaccctgatagcatttcgaaaacaagctaatgctttgtccagttcttcagtgaagacaagctcacgccctaatgcgctataggcataagcatcatttggatccacttcgagagttctctggaagaattgaatcgcaatatcgtgttcccgttgcagaccgaaacagttccctgcagcacaccaggcctctggctggcgaatttttatccatgtctgtgaagtctttggacagaactgaaagagcaacctctttcggaggatgccaaagtgttgtagagtagatctccatgccttcgactctgtaattctcaatcctcctaacctctgagaattgtctttcagcttgcgtggactctgaaagtttacaataggcccttccgatttggcacagtacccaaccggtattgcagtggtgagaagctagatggctcaagatgctgatagcttctttgccgtggtaagaacacaaagctaaataacctttccccctttcacgaagaaggctcatcaagccttccgctgctgctttttgtagattaaaagcctgaatctgaggcgcgattgtggctattttcccttctgaaatgacggaagagtccaattttgtcacttccaggctatcacttatgttcggtggagttattgctcctttattagttttacttttggttcttctgtttgggattttaggtggaaacttcatttttaattttctcctattctcctcggttgtggagctgtcactagtcaagagtcgtgaatttcttcgaggcggtgcatttgggggagatgccatagtggggctcaatacctgaggtgttgcccttgtcggcggaccagaactttgtgtttttgcaaggactggagttacctttcggctctttcccctctgcgagaagacagacggtgttccggtttggccgattctggcaacaggcttttttgaaggggctccggtggatggcacgtcaatgacagacggtgtctcataccagtgcagttttgtcaatagggtccgtctccgggacttggggtttctaatggcaaaatgccaacacttggggttaatggactaacagctgctggtcctcctaataaacttcgaccagtttttggtttatgttgaacctgtttagatcatatggaagttcctgttcccagtgggacagtatcaggtgaaaggacagctgaatcgatagaagacactggggagtctgtattcaaggagtactttgaattggaagattctaaattccatccgtttcattcgacggtgtcctggggtgtttccgtaagaacggtctcgggctgtctgtgacataaactaggacgaggtccaagtgttgtggcgcaacacttggacaggcagttgctaaagctctctagagaggtgaatcaaaatgtttggtcaggatctggcttttcccccctatttcacatcatgattcaaagggacaccagaaggaaaggatttcaacgaaggctcttttggtcacattctgatcctttggtaagccgatctgtcttgcaatatacatgtcccgacgatggaaggggaaagcgagctgaatcaccaaactcaggaacgataatatcatcgtggcttttctgcttatgaaacactccacccgataagatttgatccccttctgcaagcttgctgagatcaacacaacatttcgcaagcaggcatttgcattgcggggtagtacaactgtgtcctttcaagagtctatatgttttataggcctttcctgagcggtaagaacaggtcgccagtaagaacaaggcttcttctgagtgtacttctgcataaaggcgttctgcgggggaaaccgcatctcggtaggcatagtggtttagtgcttgccatatagcagcctggacgggtccctgcagcaccgccatcctcgaggctcaggcccactttctgcagtgccacaggcaccccc

SEQ ID NO: 11294 - RNA, 3429 nt, Homo sapiens
  source 1..3429: mol_type = other RNA
ctgaatagctgggactacaggtgcccgccaccacgcccagctaatttttttgtatttttagtagagacagggtttcaccgtgttagccaggatggtctcgatctcctgacctcacgattcacctgcctcggcctcccaaagagctgggattacaagcatgagccaccgcgcctggcccagtgtacgcctatttctcttcacctttctctttccttcttttctctctgaaaccttccttttttccttttctctttgcactgaacccccttcctctgctttcggtcagtccagtggctcccagtgaccacctatccactgctgagcccttactcagggctcctcagctaaaccacaaatatctaactcatcacgtgcaccccaatgtgttctctaatttggaagaatttcccattatacttcaatagacaatgaaacaatgtgatgatttccattatacatggattcaatggccatgcaaaatacatgacaaataatgcctcaaaaaagtttcttacagaatgtgccttattttaaaatacttacataccaaaaaaaaaaaattacagaatgaactgaaattcaggcactcaaaagcctatgatgtcagatcagcaatcacaaaactgaattccccagatcactgggaaaactgcaaacagaaaatcttgcccccaaaccatcaggtaaatctaggtattgtttactgaaattccactattttttgaaacaaagaatcttctttgctgttgttttcagtttaggatgtgtgataataatgagaacagaatgtcctggagagtaaagggtggcaaaaatcagacaaatggatttggtccccatatccatccctgcataaaaggggagatactggaccagggtagcaactgaatatggaatgtagaggatgaggaaatagaccatcagcttcatagcacctacatgagcttccgtctggggattccagaaaccagtggcatttttctgcatcttctgtatatgtctcctcaaggagtgtattagcaaggaagcagaagtcacattaatgatgaactggagagatgagctcaagaccaaagaaaccactaaagacaagatgccctcactgatattaaatgatgtgttatttctcgtagtcacaagttcaggaaaaggtgatgcctggctaagcgtgatgtacaggcaagtggtgaaagcagaaatcagcacacaggccagcagcagcctggggatctttggggagatattccgcttcagcaggagaaacactgagtgttggaagttagtaatcttcacacagtacaagatattgagcaaggtcacaaaccagacactgctcgagtccaaaaacatgaaacacaacacaaaaaaagcagacaggtagactgacctttccgtatttgaagagacgaagtagatggtgttcaccagaaatagtcccagcataagaaacctggtgatgcccaggctgaacagaatcctatcagaagaggagattctatggcttttgacccaagttttgcaattgaccactgtaataaacagattcataatgattcctacaaaatttaaaataactgaggcaataatagcagagaaatagaataaccgaagcatctttactcattgaggattcagcagttgtggtgctgatagtggaggcagaagaaataccaaaatgtataagcagacaccagtatccagccaggaaggacatctcctttttaatttttcccagcatggcaaatgagccattcatgatcaagggccacctgattttactgagatgcaaatcttccaaggattacattactatttcttcattagtatcctgttctccttagaaatgcctaattacagcaagcctaggtgatgctgggagtccactcctccaagagcaggagggcgagagggaagagtcacagcaggctccaaaaacttagaatccaaaccagagagcttgagtccagcaatgtttctgtcaatgttttacggtaaagtttttcttcataaaaatgccagaatatggtggaaatcctaattcctcactcctacccacccacctcctagccacatattcatggatgaccagaatccaatttctctctcccctctaatctgttgctgccacaacaagtttcaccaattggccatgccaatgccactctttcaacctcagtgattcacctatagcgatttacagtgatctaatagatcaagttcaaagacccaatacctccttgagaaaacctttctcaattaatcccattctttctgatgccctttgctttgccttctctatctacatacatagatttgtgccataaccatttgctatgttctggttttccttagaaaaaattaagtcagcccttgtaggtgtttcctttataaatctgggtttatgtttagatcatatgtggctattttctcttaggcatttaactgtcaatccaggtaccctggaatgagatacacagtaatgcattagttgtagttttgtgagccaaacagctaggcatctcattgctggatttctctgtacttgctcagatgggaaatggcaaaatatccctggcaaatgatattatggaggcccataggtgaatgtaagagtatggcatctcttatcttctctagcagctgaatgaaaccaaggtgcaatcctggatgcagccacagatgttaccaaagtagcatcaaggtacagcacaaagtcctactgccaagtccaaatagaaacagacaagaaaaaggagctaagatttaataataatcaggtccagaagaggggaatacattcatgaggccctttaagacagatgacaggaagcctagcctggagaaattctctgacctggtgcccaggtgcttacagaagctttttattcaaaactaacaggcactgatagaggcatgcccacatcaggtaagcaggcaaacagaatgagccaggaagactatgactaaaaggaaaattatagcacagatttccaattacttatccatagatggctgcattaaagtggtgaagttgaaatattactaacatcacatttaaatagaataaatgatatagagtaagccataacagataaatgtggccaaaagagcaggaatcccagaattagatagtaacaaactctatctagaatgtactataccaaattgttgggttctctgtaggaggaagtgctataattaagatgtgataaggttggctagcacaatcaatgaatgagctcattcagttagaagttatttccacaagggtcagtataggaaaagtgttagcagaaccctttctccctatgcatgagaatttgacctatggttaaacttcctagctgttttccttatcatgatgataaggatgataaggataatcttatccttatatgataagggtaagaacatcaactatgtttctag

SEQ ID NO: 11295 - RNA, 11209 nt, Homo sapiens
  source 1..11209: mol_type = other RNA
ctgaatagctgggactacaggtgcccgccaccacgcccagctatttttttgtatttttagtagagatgaggtttcaccatgttagccaggatggtctcgatctcctgacctcgtgatctgcccgcctaggcctcccaaagtgttgggattacaggcatgagccaccacgcccagccttcagtctgtttttgttcaaactgtggagctgcagattaaagttattccattttagggaaaatgtccaccatacatcctacttgcaaagactatcctctctgtcaaacctgtgagccaattctgaccttctaacagaaaaagtctgattttatttttccattcaaatcaatgtggttaatatgtatcctgtgtcaaccatctcactttcagtttaaattcttctttatttctttttttagagttaaggtctcgctctgttgccaggctggagtgccataatgtgattatggctcactgtaacctcgaactccagagttcaagtgatcctcttgcttcagcctctggagtagctgggtctacaggcgcatatcaccatgcccagctaatttttatttttattttattatttatttatttattttgagatgtagtctcgctctgtcacccaggctggagtgcaatggcatgatcttggctcactgcaacctctgcctccagggttcaagcgattgtccttcctcagcctcctgagtagctgggactacaggcatgctccaccacgcccggctaatttttgtatttttagtagagacagggttttgccatgttggccaggctggtgttgaactcctgacctcagatgatctacctgcctcggcctcccagagtgctgggattacaggcgtgagccaccgcgcccggcccatgcccagctaatttttaaaattattttttgtagatacgggatcttgctatgttgcccaagctggtctcaaactcctggcctcaagccatcctcccacttcagcctttcaaaacactgggattataggcatgagccactgtgtctcacctgaagttgaattatttttaaaaatttttattattttttcctttttaatatatatttatatattttacaatataacatgtcaatgaatttgaattcttaaatgaagaaggcacagaactgagccacagggctgcccctgtgaactttctcaaagaagctctccaggctttgctctttcaaggacttcctcaagcagagcattctcaagtggcccttttatttgttttttacagcgcagagcaaggagccagagtaggattcagaatgagggaggggaggcaactgggaaagtggaagttgggaaggacagctgtcaggcctgtggcttcttaggcccaccaatataaggaggggaacatatggagaaggcggctctggaaactgattactttaaaactatctgtgtccacctaccttctagaaagtcttcatgtccttgtaggggagtgcaaaccctcgtgtgaaggcctctgacaccaagtgtgagaagccattgatggagccattactgcttccttcgttgtagcagaagggatggggagaggagcaggcaggagcgggggtaggtaagttgtggctttggtgccttgaaggtgaggaaatttctatttgaaggcttcagttttcttcatgaagaattttttttttttttttgtccactgaggggtgggggaaggtgagatatttgaggaaggtggagaaaatataaaagagtcaatacaaataatcaaaactagtagctagaatgaatactagctaggcagagctgagggtccagttaagataggtggtcatgaattcaaatctacatcaatctgctcagctgtgtgattttctttagcaatattaaagctcttgtttgtttgatggttgtggatttggtaaaatgctgatctttcccctatattgagaaaaatgtgagtaatcacaaagaggcccgataataattatgagaaatttatcaaggcccttccagtgttcctctgcataaggtggctttggatggccagacatttacatagcacatagtggctttcttttgtttctcatattcctggtgaattgaactacgatttcttctcctaagcataaatacctgcagaccttagttacagtcatccctgtgaacaagggtgtgggtagaaagggtgaggaatgtctgtctttcctatcaccaggtaaatgggatcttgatgcttggcatggggtcccaagagcttgccattacccatgtgtattatcaaaaaatgagatactgccaccgtcaaagaaaagatcagggccgggtgtagtggctcacacctgtaatcccagcactctgggaggccgaggtgggcggatcacaaggtcaggagatcgaaaccatcctggctaacacaatgaaaccccgtctttactaaaaatacaaaaaatttgccaggcgtggtggcaggtgcctgtagtcccaactgctcgggaggctggggcaggagaatggcgtgaacctgggaggcagagcttgcagtgagccaagatcgtgccactacactccagcctgggcgacagagcaagactccgtctcaaaaaaaaagaaaagatcagaaactctctggacgataggcaaaggttgtaaaccaatgtatcctctttcttaaaatctgatttaaagccttcttccctgtcctgacatgcactgggagaaggacagaatgagttggagggggctagggaaattttggcttataactctcttgagaaatgtctttttaaaaattgtctcggccaggcgcggtggctcatgcctgtaatcccagcactctgggaggccgaggcaggcggatcatgaggtcaggagatcgagaccatcctggctaacactaaaaatactctactgtctctactaaaaatacaaaaaattagtgcagtgagccgaaattgtgccactgcactccagcctgggcgacagagcaagactctgtctcaaaaaaaaaaaaaaaaaattgtctcaagctggaatattgcccgcatatcatggtatgggatatgctatatatcagtaaaatctaagattcagccaataaaatcagtctgtctaacactgtcactctaaaagtccccaaatcaccacagccatggaaggatggttttcccatggtaacagactatatcaagtttacatatatatatatatatattttttttttttaagatggagtctcgctctgttgcccaggctggagtgcagtggcgcaatctcggcttactgcaagctctgcctcctgggttcacatcattctcctgcctcagcctcccgagtagctgggactacaggcgcccgccaccacacccggctaatttttgtatttttagtagagacggggtttcaccatgttagccaggatggtttcgatctcctgacctcatgatccacctgccttggcctcccaaagtgctgggattacaggcgtgagccaccgtgcccgacttatttatttatttattttttgagacggtgtcttgctctgtcatccaggctggagtgcagtggcacgatctcggctcacttcaacctctgcatcccgggttcaaatgattttcctgcctcagcctcctgggtagctaggactacaggcatcccccaccacgcccaactaatttttgtatttttagtagaggcggggtttcaccatgttggccaggctggtctcaaactcctaacgtctagtgatccacctgcctcagcctcccaaagtgctgggattacaggcatgagccatcatgtccggcctcaagttatattttaatagcatacaggatacatactcgtactcagaatgtgagttcaaggatcagtggcacaaataggggaaatgacctcaagttccaaatgttaatgtagttctattagagtgtctgagtggggagaaatcatttcttgaattttgcagggcaagcataagtgctttgactcatttttgtacgcctcacagcgtgcttgtaagccatgtctccagggccatacactcattgtaagtgcccctaataataataaagcaaaggatctgctgcaactcaaaggaaataggaagtgctttaagttccacattccaaagtcagggctagagaggcaggctggatttcctgctgatgtggattgcctgctgttggtttgggccattctaggtataaggtaatgttttagattactgctgggttcttctgggcctggcaacataaagaacaaatctaatcaatgcatcagctgctatggctcattcaccttcctgaagtgttgtgtggccacagcctgcaagaatatgacctggaaatccccaggtagggccctcgggtgtgctcagatccctcatgcccacccatccacccctctgcattctaacatttcagtggttatgttcaggcaaagtgtcttctgctcatgcttgggaggaagagttcccttaacctccctgtggctcattgtccctgaggataccagggctctctcagcctggctgcatgatgacagagggacaccattatcagagaaaccagggctgatgagcagctctaggtcagagaggccgaatgctacctggacatgaagagagaggtcccagcagaccccctggggacaggttcaaattaggttccagcttccccttcctggtgtcaggagttactcatcttgatttacttatcttgcaaaggagccaaggtatcctgccgtacctgcctattgccttctgtctcttccacaactcccatgtctcttttcggtttctgctccacttctcatgggctacttggagtaggaagtaggtctcaataataaaaaactaaataaaacaaaaacatcatctgatttgcctccagctctgccacagactatttggccctagaacaatcccttccctttcctgatactcctctgtaaaatagcctggatcagtagctttcatattacattctgtgaagctgccaggagccggaggggttccccagatacccggagaggctgcagtggaaagacaggctaagctgactccacccccaacacccagcgcccaccagagtagctgccttttacctgttttatatattgtttttccacacagagcttctttgaagaaagagtcctgaggctacaaaatttgaaaactgctggaataaacgatcgccaaggccccttccagtctgagacgcttggtcttctgaagcccagctcaagtttttcctcctccagaaagcctttcttgttacccagtcctgggtacttgagctccaacaataatgatgatggcaggcatatggtgccgtccgtgagccatccgatgcctgcatgtgtgcataagctgtctccccagctagaaggtgagctctttgagggtggtgttcaatttttcttccacacctctgtccccttgtaataccatatgcaaagtaggtgttcaataaacatgttgatgccacctggtgtcatgagctctcacatgggataaaacttccctaccaggaagtttgggaaggaggaaccagcctttggtctgcttaacgctccacagagagacttgtccttaaaaagctggggaccctaacctgggaagcagcttcagactcatacacttcccaaagggcaggtctgagttcctgccttgattggatttggcttcacctcttctgcccctcagtacctcttctggtggggcctcttatacactgtggctgtagaagaggcacggtcctgaagcctgggaatcaggtcagctaggacgccccagggccagcagacatctcagccagattccagagggaggcacgggggagatggagaggaactcctgggtttttttggaatacagctctctcaggaagtggaggcccaaagagggtggctggattcagtcagagacaccagagaaagcagattggaggagggtgctagcggtgaaagaaggcaggtagccaaagggaaactggaggttgtagtggtggaatgaaaccgctctgccatttagtggctaagtgaccctgaggtcagttcatcttacttagtctcaatgtctttacctataaattgggtgtcaaaagaacctgaccaatgtcaggctaccctgtagtgaagtagtgagatagattccaaggagactaaaatgtgcagagatggaaaggattattactgtttattaacacaggaaagcacaggagcctgcttccaaagagggactgtcccgtaattgagagatgctccaaggctgaccatcctccttctcctgctgcacacccagcagccatctatggctggatttggagaatttctggtcaaaccggtgagtatgaggagagcagggcagttggggagagaggtcccagcccaattctgcccagagaagctcccaaaagagagggaagtgtcctgatgaagagcccatgaaaggggtgagacccaggaggctgtggagattgctgcgggctcctctggtcagtaaggaaccctgacaagatccctaggatgggggtcccttagtctcactgaagttcttgtaacttgggatgggggccaggtcagcctcctctgatacccgaagctacacatctggccttccccacttctagaggaggggtcttagatggtgctgtgggagcagacaagccctcagcaggtcgcaagcaggtcccctccaaaacccctcctgctggaatcctccagatgtgaggagtaggagcagacagatcaaggctgggacatctggcagggtttaacatccacagctggagggtgagacctctccctgtggatctggagaaataccttcgggctccagcctattgctgcccttgccttgtcatccatgacagggttccgcgccctgtccagcctccccgggtccccctcagctgctatagcctgacgtgtgagtgctgggcctgcgcagccaaacatctggcaggtctggctggctattgggcagcaccacagggctgccatcccctggcccccctcggcccttccaggacaagctgctgtgatgggaagcgggcaatgatgggtcatacactgtctccctcagcgccagccacagggtgtcccgcttcccattgagctggcctcgctcaaggactggctgcccagtgtcatccaggtcatctggggacacacccacggaatctggtacacgggcactgggctcagaggtgcttaggcaggtctcatcagagacgctgagcccctccagggtgctggctgaggaacagaagccatcaggaggatctgcagccttggccttaggagagtgggctggggcttctggtgaggctggcaggggctcagcctcctccccttgggagtcctgcctggcccgggttttggggctggggccagcctgcttatagggggaggaggtctgcagggcagggcactggctgaagactgcctggtggtccagcagcagctcccttggggaggcaggggctggtgggggccgggaacagcacggaccatcatggagctgcagatcctcagagagtactgagggccggtgggacagcttgctggtggctgtgctggtgtcaaagctggggctccgacgccgtgccaggggctgtagctcatattgctctgagcaggacccgggcatccctcccactgaccctggtcgtgggcggcctgccttctccccaccagggtccccagtaccagcatcccatggcaggtgggcacagggccagaggatctgcccacagttcttctctggcccgaagaaacagcagagagattggaagaagaagctggcaaagccacaactgacgcatttgaccatcatgaggatgatgcccagcttgcgatagagcagcactgtggcaggcagcatgagcacgcctgccgcaaacagggctgcagcccccacggctgtggcgcagctggtctggcgcagagagaaggccacacggctcaggcggtcagggtgtgggcacaggtgataggagatgcagtagttgacagtgaagtctactgagaggcccactgaggcagagagaaacagggcctcggcagtgttgagctgccactcgaggagaaccaggagtcctacagtgagcagcacggtgcctgccacagctgccacggagaataggctgaggggaacattccaggtgcccaggagcagtgtggcaaaggccagcgccaaagccaggcccagcaccacagcaggctcagtgctcaggctgtgctgcaggctatacagctctagacggctagtgaaccaaccacggcggaggcctggaggtgccatgcccagctccgctgccagccagtggctgacctcattgtagaagagctgggtctggttgtagtccggactgttccggaagttggtctggaattgtaggaccagggcggccaggctgccatgggcatcaaagcggagtcccaggtcctgggtgccatcggggccttgctccagagccatcattttcaggcagtgcaggaaaaactggggggcccaggggaagtccgagtggccgcagcagaggtcaggccccaggcgggcgcagctggggctctccatccagcgctggagggtctccacgaaacacagcgtgggccagccttcctgcagggtgtcgaagaagctctgattccgggcccggtgacagagtgccagcagccagcgctgggcctcagggccgctggccgagaaggcagggtccctcaccaggctgctgttgctacgagggtccagagggtcgccagtgtccacaggcaggacgccccacaccaaaaccacgggcatgtggccgccctcgccctgcggcagctgctcgaacaggaacagctggcgatactccgcgtcgaagcgctcgaaggggtggctgggccggaagacctggccgccgggcggcggcagcgtgggcagccgcaggcgggggctgactccggcgatgtaggcgccccctgccgccagtgctgcgaaccagcagatccagatgtagcggaacttgatgacgccgcagggcagcaggcgctggaagagcagacgcgaggtgccagccgccgccctccgcaggccgcggagccgccggtgcagcgccagcagtagccgccggggcgcgctgccctcccaccggccccgcgcccggcgcgcacagccgcgcgccaggtagcgctcgtggagcacggcggaggcgggcagccagaccagcgtgagcgccaggtgcaccagcacagccgtgcccatgaagagggcgaggcagcgaacggccggcaggcggctcaggtagctggcatagaaggccgcgctcgtggtgaggccggagaccagcagcaggtagccgaagtggtgcatggtgcggcccacgcgctgcgccagcccccccgacggcagctggctcttgctaaggcgccacaggtcgaagaagatgagcgtgtggttggcgcagacgctgctcagcaggaggagggctgccagattgacgaaggggaagtaggccatgcggaaggccacctggtaaaggaagaaggccaccagcagtgagcccagcacccccagcagcaccatgagcgtgaggaagagtgagcgcaggtacagggccatgccgaagaagatggcaaccagagccagcaaggggtacaccgtgtcctggaccaggaagtgcctcagcagctcctgcttgaggcccaggtccatgccagtgacagaggtgtagttgtcagcaagcccccagggggtggccagccggtccaggtagatgtccatgagggaagcaccctttggggtgggcaggaagagcaggctgtacttgagggaaggcacctggtagtcagtggtctggggactcagaaagtccctgtcaagcagaaagtgcaggagttggtagatggcactactctgggagcacttggtgggaacctgggcacagcgtggggacttgttctgcccaggtcccagacaagagggcaccaaggcgccactgtggtagtagagggcacaggtccgaagcagggccagtgtgcgggctgcgtcagcttgggtagtgtccaggcaggaggagcggttggagagcacagccagatagttgcccagggaccagctggggcagcactggttggctgctgtccgctggcacagagccccgaagctggtatgggagcggatctggtcctgttccatgcgacacatggaatggatggcatgcaggttccataggctgcccgaggaggtggacatgaacaccagctttgcatagctcttctcaggggggccacagaagaagttctcttgccttctgtcctccaggggctccaccattctccgaggccggacagcgctctcctgggcactgcctctgggtgcaggcctcagagtgttgtgggagctcgagctgttcagctcaaggtctggggaaaggaaaagcagcttcctggggcctgtgagggcttgtagtgctctccagaccactaacttgctcccaatgtctgtgtcccgtggctcaaagcccagcaaaggcttggagaagtcgggcagccgggcccccaacagtccagccagggtgcagaggaagatgacagccagacacagcatcagcacggccactggccactcagcaatcagctgggaatagctctttggcatctggaaggctcgttcctgcctgacgctgaccacatggtgctgcacagcgggtggcttccaggtcccatcgcgctgtgagggggctggagaagggctgaggctggagccgtgggagcagagagctgcccgatccccaagtcctggcagggaactgcccccctggtattcctgcagtgcccggggataggtgaagtgggcaggggccaaggggctggatggacccacaggctggagggtggaagttgttggtgggggtcctgaagagctggaagggtcctccagggggcagctgtggagggagcagcttctctctgggcttgcctcagggggcacagccttggtctgggtgctgtccggggagccgccgtctggggccaagggctccccctcgggccgttgctccccttccggacccgggccgggagccggaccgctgccgccgctgctgctgctgctgtcaccgtccatgcccgtgggcggcaccgctgtccgggcgctggtgctgaagccgcggcggcggcggcggcggcggcggtggcggcggcagcggcggcggggtgctcgtgcgcat

SEQ ID NO: 11296 - RNA, 4490 nt, Homo sapiens
  source 1..4490: mol_type = other RNA
ctgaatagctgggactacaggtgcccgccaccacgcccggctaatttatttgtatttttagtagagacggggtttcactgtggtctcaatctcctgacctcgtgatacacccgcctcagcctcccaaggtgctgggattacaagcctgagcgaccgcgcctggcctgaaaaggacactagtaaggaaactatgtaattcagtgtttctcatttgaaacattttgaactgattagtcttttgttattagaattgattatctacagtgttttgttgttacaattgaacattcctagagtttgcttgctttttgtaaattactccagatagcaatttaggaaactcctcattatttttgtttagggctaaaatgattctcctggagacagagcagttgtacttggggtacaaggaagagctgtgctgaacgtcagccagggaaccttctaagtcaccgctgtgggctgtgtcctgctgtttatttccttaggttggagcccaagtttcagcataggtcacctgttaacatctttctctttgataagtcatcaaagagacttgggctggaatatcctgccaccagggggaatgttcaaaagtacatctgctccagaggtcctccagtgttgacaggcacattgtagcaaattattgggttatacagttaacaaataccttttgtttggagctgtaagacccaattataaagcactagtagtttttgtctttttaatgcattaacaaacatatattgcatgtttatggtgtgttctgcattcactaggcagtggaagctggagctaactagagcacagttcctgtcttcagaggtcagtagcatactggaggagatggaaaagattgaatgaatcacagcctcatggggtacttgagggatgatatgactatttctctgcatagcatatctccattagagcactagtccactgtgtaacaataaccttgcatacatgcctgccacttctaactagtgagtccttcctgggcatgaagcacgtatcattcctctgtgtactgcagagttgtagacactgtgcttgacacatagattttagtaaatgtttatgggtggaactaatgagagaactagaagagggagtgaattgaatgttcttgagttaatgggaaggagttaatgaaggcctcacagaggggcaaatgagctggatcttgtaggatctgtaggagtttaccaggtagagaagagtgactccaccagcaaggtgtttgggatttctatagttaattgttaagaatttattcctgttccccagatccttatgactaatgccaacactaaacataaaacaggatgttactctttctacaatgagctttggtgtttttgtttttgaaaaatattttcggtatatggtttttgtttctgataggaattctcctttaggctattgtcaatttgttttcctgtaatgatttgaaacaattatattaacttaaaatgatgtcacaatgagtgaaataatgaaaaaaagttatagttattgagggtagtctcatgatgagataaagtgcatacagctgcactcatgtcgccaggtgattaagaacagaattggtattaaggtcaacggattagcaaaaagggaggagattattgtcttttcattattttgaaagaagtaccatctgcccttgattgttttggtttaggttttattcagcccaaattagaatccgctgtggtgttgattgttccttgttggtgatagccctagaactgtgtttcccatcgttgatacttgcattcacgtttgctagttctctcttctcctgtgaagacatgaacgtagctgctcctttaattacatttagctagttttaattcagagatggctattggccctttgttttcttaccatcttttattgtgttcattttcctagttgatttttaatggtgacatcactaacagctctaaagactcaaagcttaccagacagcacgcttccctgggtcagaagatgagagtcctctcctctctcattcagtaccagggtgtaccagtgagaggcttgtgaagggattgtttcggcgactccttatctaagaaatgaagataatttttatgaggtgcattttggtctgtgggagtggaagggaaaatgacggtttctttcctatactgtcctttgtttggaatggtgaaaatgttttgaatctgtttctggtgtgatcgttaggtccaagatttcacgtgacgttgtgtgccgggtgttgtggtcaacacacaggaatgctcctttattctctgtacggcctttgggtgcatcatttgagtggatgttcatttgcttgagacgattgtcagagggaatcttgtgtgccctttgctctctgtgcctgtcattgcgagggtttctttgagccggtctgctgaccgtcaggcacttgagattgactcggtgaacaatgccgccagcctttctgatgcggctcctgccctctctgactcctacacaggatcagaatcactcagatatcacttctgttggtggaggcgagagaagaatatttatccagtttctgcctttctgcccccattagctctttaccaaaaaaaaaaaaaaaaaaaaaaaaaaaaaaaaaaaaaaaaaaaaaaaaaaagcaaaaccagttattctgtgaaaatatgcaaagcagagttttggccttgaggatgcgtatttgtgacttgctttcctgtacagtaagtgctgccgcctcaggagcgggcgcagtcgcttatggtgccggtgagcctgcgcggcgctggcttttgctcctctggtgccaatgcagctcgttgacagctccaagatatttggatatctcactcttccggctatttcagctgccaaactagaatcccaaccttctgagagtctgttctcttttggatttgttcatagatgtctattctctcctgatctggttcatgaacactctggaagccaagttcattgaagacactctggatgtgtaatttggaagaggagactggagcatggaggctttgttcctggtgccatgctagagcgggagaggagtgactgcaaacctaggcctctgtcctgtcacctttcctccagctggtgaaccaccttgtctactcccttgccccaacacagccgacaggtggacagccagacacatgcagagccattgttttttcaaagacctcttttctgaactatagatgggaagctgctgcaaaaaagcaaggtgcagcccctttcttgtatgagggaagctactgtttaccatccatggctgcttgagtttttagagctgcgtcagatgaataacttgttggtatcactcgtcaatcttagaggcactttcagagattaggaattgtgaccaacaggagagactatctggcattaggaacaccagggcctattttggatcatgctgtactgcttacggtcatgccctgtccaatctgggatgactgtggcatacaagtcaccatggccattgtgaagcccttgttcttggagaccctgtgctccaggtgtggctggttggttccctgtggcaggacccccagaggccccaggggttgtgagagtcaggggtgtgcaggttctgagggctttgctgggtgggccgaggttgagtgggctggttgcagaatcctggtgcccagagggttcttctttgcctgttgctggggactcacgccttgtgaggggacctttctttattaccctgatgaggacagaagagttcctgagaggaagccacaagccgcctccctgacctggcagctgcctgtgtgccctggtgtgtgggttcctcccttcctgggttcatgcagcagactcttggcagtgcaggcctccttccaggggctctcagggctcagttctcatctctctgggtcacactgagccctgctgatccccctcctgtgtggctgcctctctgatgcctgaaacaccttcagctgttagtcccacggcctctcatcacctcgatatccttttctgcttgctttctggttttcagtggctgccagcagaggctgtaatgctcccctgggacctgaccagtagagaacaaatgctatgaagaccagaggcccctcactgctccacgcgtatacagggtgcgtctgtctggacagccgaaggcccatgggtggttttgttttcaaaacacaatgaaaaatgactagtcatgccatattgttagcacctttcgattttttttactgtaaaaatcaaaacagaaatatttggctccagagctctgtgaaccccgaaaatttgagacgggtctcagttaatcttgaaagtttactttgccaaggttgaggatgtgcgctcattaacacagcctcaggagatctaacaacatgtgcccgaggtggcctgagcacagcttggtacgttttagggagacatgagacaccaatcaatacatgtaaaataaacattggttaggtccagaaaggcaggaccac

SEQ ID NO: 11297 - RNA, 665 nt, Homo sapiens
  source 1..665: mol_type = other RNA
ctgaatagctgggactacaggtgcccgccaccacgcccggctaatttttcgtatttttagtagagacgggggtttcaccatgttaaccaggatggtctcgatctcctgacctcgtgatccgcccgccttggtctcccaaaatgttgggattacaggcgtgagccactgtacccggccacatgcaccgtcttactctccctctgagctgccacccaactgcagtcacagctgtggccccttctctgtctagctgaggcttgacccaaacaagaaacccccacatctctttaccttagtccctttaggatgtcaccaagcccacagcccagggcaggcaatctgtgaactgaatgaaagtgagtggggtaagggtgacagtgagaacgctctgctggccaggccaggccggctggaatgctcgaagtaactgtttaaaaaaaaaaaaaaaaaaaaaaaaagccctagtgggaaaacgatggagaaacctgagtaagtcacccagctgacaaagcccagctccggcacacataatagtagccatatggcacacacacctaatagtcaggtccacttccacttccaggcgggagccccccccccccatctgggaactgccagcagggatcccaggccctccccaagcccctgctcctcccctgtgccgg

SEQ ID NO: 11298 - RNA, 2102 nt, Homo sapiens
  source 1..2102: mol_type = other RNA
ctgaatagctgggactacaggtgcccgccaccacgcccggctaatttttgtatttttagcagagatggggtttcaccgtgttagccaggatggttttgatctcctgacctcgtgatccgcccgtctaggcctcccaaagtgctgggattacaggcatgagccaccgtgcctggccttccatgttgcttttttaaggctagtcaagtgaagcagtgggaatgagaaggaacacagaaatctgttaaatgattgtgatcaattggttgtaaacatcactgcacttggactagcctcgtgtcattttttaatggaaacatgatttgttttcttcttgtcatcatcttaagaataaaaagagtatttgacctttgctcaaaataattttctctttgggttacaatctgaagggcattaattatgaagatattgttataattaatgcccactgtctaaaggagaattctcagccagttcagacctaaagagagcaagatgtcgtttgagctttttcttctcctctgtctgttcacacaatttgacttcaatgttgccatcactgaatgcttctcctttggtttcctccactggattctctctgagggaaaactttgctttcttccgcatcattgtaattcctgaatttccatgcctttgtgctggagagaaggttttatttactatgcaataacaaactgcagacaaaacattttttttgaagttttcattcataaatgcatagacaatgggattacagatggagttggaaaatccaataatttgcacgatagcaaaaatcatcttgattgtgacatcatcatattccttttcaaaattactgtattcaatcatcatatggacaacatggaatggtgcccagcacacagcaaagagagccaccactgtcaccatcataatgacagctcgtttcttcttcctggctattttggacatttcttttccatgaatagttcgaagcactgaaccatccccaactcttttctttatccaaagttcataaccaattttactgtacagaataagcatcaccataagaggcaggaggaagaggatgacaaggatgaaggtggtgtagatcttctggtgcacagggctggtccactcttctaagcagcagatgtgttccttttcatataggaagtcatatttgatctcaagttgttgcacgtgccacatgggtgatcctacgatgactgccaccagccagaccacacctagcattgtgaaagcccttcggttggtgtattgccacttcattttaaaaggatgcacaagtccctggtgcctttccacagcaatgcaggtcatagtgaggatttctgtcacaacagcggtagactggacaaatggcaccatcttgcaaatgaaagcaccccccagccagttgtcggaaatgttctggagcatggtgacgggaatgcagaagaaggtgatgagcaggtcactgagcgccaaggagcagataaagatgttggtgacggtgcgcatggccttgctgcgggtcaccacgtagaacaccagagcattgccaaagagcgccagggcgaagatgagcacgccggtgagcacgagggccagcttggcgcgtcccggcagctctggggtgtagacgagcggtcgcagccggtacagagcgatgaactgctcccgcgtcaggttgtggtcccgcagcagccgagagaactgctccggggtaatgttaagcgcctgcattgctgtgcgctcccgggacgcggggccaccgcccgctactggctggccatccgcatctgcggggcagcgagggcttcgggggaccagccggaggccgcctcccttcctctactctggagtcagccgcgcgggagggctctaggctgcaccccgggaggttcgggaaaggagagcagctcagggatcaaacccacgataaagaggcgggaagccaaagcactgggagactcgatctcagtgaccaaaaaatgttcgcggttcaaataaagttcttcccttgctcttccctaaggcgaggcgccgccacggtctggggtgctggagcgccacgcgagggtcctggcgcctctggctccccgccttctggccat

SEQ ID NO: 11299 - RNA, 7001 nt, Homo sapiens
  source 1..7001: mol_type = other RNA
ctgaatagctgggactacaggtgcccgccaccacgcccggctaattttttgtacttttttttttagtagagacggggtttcaccgtgttagccaggatggtcttgatctcctgacctcgtgatccacccgcctcggcctcccgaagtgctgggattacaggcgtgagccactgcacccggccgccaacaggtacatttctgtattgtctgtacaatgttaaaataaagggaacagtagtttctgctttcttgcttgctacctgcatgcaattgtaattcctaccttgatcagatctaatactactgacaatccagactttttatatgtgatctgattcacgatcacatatcctaggaattgaaagtaaacactgagattctgcccaataatggaaatagtgttatcaaccatgtagcatgcaatattcatgtagatattatccaagtagcattttatatgcttgccggtaactctgagatagaatgaataatctttcttgagattactagtgtagattcaggtcttcagtgccctctcaacctacattcacatgaatttcattcattttgaaattacagagggacaatcatgagagatatgggaaggaatatgttggggagggggggcagtctccactcacactataatggaagaaaaatgacagccaagttaggtttagctggaatctaacatatacagagctttatcactctggaggcacattttgacataataataactactgagaaagaaccacttttatctaggtcagaatgacagacttccaagtgttagagagcttgggggaaccacagtttgaaacatcaggaagaagactgcaatctgtacagagattttcatcaagtctccacactgccttatgttttcatccaatacattgtaattactccactggcttataatggcgtagcattttgatttcagagcctaccaaaataaaataaaccacactttatgacgactacatttataataagatgcagatggtaaaggaaacagatgcctctgacatcatctcccatttgctttcaacttttgcagacactggcagtctgtaaactcattcaaagggatgcaagataagtcaggcagttttccaattctgtttccagtttaaaaagacactgcagtggcactactttgagtcacagagtgttaattccagaaaaataaatttgattctaagtctgtgtcagtctttaacgcaaaattaatcaactggggggaaaatgccccacaatattgagagttcagcgattagtaactactgattgttttgcttgacagtgacagaaaggataggatgggagtgatgtgatggcgaacagctgtagctccagggaggataaaaagtgaaaggagagttttaaacagacaatcatgtctaaaataatctaccagcccttgccacccagattgttcaaagacttattccttatatttctaagtaaaaaacttcaaggaggcttttaaagtcagtttccgacctcaaaaaaacatattcattctgtatttccatctgtatttcccagaagaaatcctatagttctgataggagctttcaccatttcctcagtgatatcactgaacattaaacacagtaaaagaaattttctttttctttgtgcaagataagtgtgtcagaagaccttttcaaaaggataaggaacttttgtagtccatcttgaaagcaagagatgcgtgggtaaagcagcaattgcaaggcctttagcagtgtttgaggtctctagatagattagcacagttacagatgaaggggagttagacaaaaacttaaaattttcccatctcccctgaccccatgatataacttcatctaccactctgtagcagaaactttttagcagacaaaattttcagaaacaaaggcaagggaggtgatgacataaaaataaatcctgctaggccaaatatggtgccattttttaaaacaatctctctgtgcaaacaacactgaacacatacacgcgtgcacacacacacacacactaaagaataaacaaactcttctgattcatatccacaaagtgggttggtaagtattattagtgcaaatttctgctgacctgcagcatttagtccataaactttggatatcctaggcgatccatcagagtccagcagatgttttcaattagtttaatttcatctctaggcaagttctgtttccaaacattagtattagttggtgatatttccccttcatagggaaggtaaaaaaggtttgtagaggtggcaaacaatatttggtttaaactagcaggagacaaaggaattccaagaaaggcaaaaatcctttcagtagttttctgaggaaaatgcacaatatcttcaaacttgaccagctggtagctagtaggcagcaaatctgtatttattctcaaggctgctgctgtatttgctagccacaagtgagacaagagggacactgcatttgatttggattttgataattctttcctcaatggttcatactcgaaagcataacccgaatttaagttacatttgcctttacctccctctattttaaacaattttgctaaatgctctggtacattcttcaaagaataaagacttggtttactattgtacaacattgaataaatccatgcccgagggtctcttactatgtacaatgccctcatcgaagctcctaaaacttcctgaaaaaaatgaagctttaacgtccagcttccactgcttaaactgagcacaggacgtgcacttggatagtaaaccaggtgtctcctcaaagccctaatatattcagcatctctatcaaaggcgcctttcatttgacttctttgttctggcaaagactctctccttttaaattttctttttttgtccttattcattgcaaaatattgggccagtttacccctattgggttcatgcagatggatgttttgcaaatgtaattttgtgtcctggactaaagactgcaaccagcctcggagtaaacgaaaatgcccactgcggatatctgacaccttccattcacaagcatctacaaatgagtcgatttccaactcagtttcaggaatatcaatgtaggctgtaggaaccctgatgtagagaaaatcactactgttgaaaaaaagttgtttgagaatttcagctcctgaaccaggaagtgaggtaatgacaacatcaggaagatccatgtggtgcccttcagaagacaaagacttcttgcttccctcagcctctgtccttgtccattttgcacaaatgggctgactacaagtgctccacacatccaaaagctcaataaaccacaaggcaataacaagtattaatatccatcgcattagttttctaaaagaaaggtaaaaacgccattggaaagttaaaatcaccaagctaatgcacaaaattaatccaactgctatattaaatttaaatccaaaggggaaaataatcctatcatgtcttacaggctttactattgcttgagtgcccaaaccaaatcgggttatttggccttgatcagccacactggcaaagccaccgaatcccagataattgaatcttgtcttcaggttatggtaatcagttacaatagaaacaacatgttcagtattattgacattgagagaaatctgaagtccaggattggaactatcaataaatctgcagctggagacattgatatatggcccataaaagacatatgcaattcttgtgattgtgggttccatctgaaaagtaacattaacaaattgagtccatcgttttttaaattcagcagcttgctctgcttcctgtatactggccatgggactattgccatgatgatcaaaccaaaacattttgtaatgtgcatcccacacatccatcatggcaccattatacctattcataaacttatatgggatatatttaaaatcaatatccaaattatgaaagaaggcactgacagaatttattggggaatcttcttgcctctcaatatgatcaacaactagcagagtttgggaatttaagagaagcaaagcacgatatacacttttcagtctcattgctgaagaataagcagacacggcttccccactcacaaataccatttccccatgttgagaggcagtgattatttccccagctgcatcaccaacctcctcgccagtccacttaagccactgcgcacattctcccagttgaccttcccagggcttattacactggcttgagggtgatggagcaaacaccaatacattgttaaggtggctcaacttgggtccatagagagcttcagaaacaaatacttgtccattgggggcaaaagtaaatgagttctgatctggatgctcatgtcctgggttaaaacttctccacccatcaatccaggaatatggctgaaaatgaactatgtcatacacagctcgtccccccagcttcccagatttaaaagacacaaaggtgttggtctgtgtgtttggcaacccagccccataagtaaccacaccccagttagggaatgtgtgtatttttgcagtaccataatcagcaggtggctgtggtgtgagctggggatcataccagatgtattcagtgtgaagagtactccacctttgggcagttgaaggaaccatcggtccatctttaggtcggtgctttctaatttgctgagctaaccaatttccagctccattctttaagatgaacttatccaagaaaactagctggctttctggaccataaaaccaattataattggaatctgctatacccacagttctttggaagccaggtaaaagggtggcataatagaaccaaaagtgcatctttaaccagttattatccaagttgttgatattaaaatggcgctgggccagaaaaacatactgtgtgacggatttagctgtgtagcttccataggccacaccttcatccaaagaaccatcaacaatatgattcaatagaaacattgtcttttccatgacatccactacagcctgtttccatatatttgctttagatcctttatctactccagtcaccaaggcccctgtgagtaatgctatcatattagtggcttggtggttatggagaagctgtttgccccatgagcggaccttggaatactcgtacatttcctcagtaataacccatattttttccaggtatttttgtcttcgatgattatctaataagttatataaaaagtcaaaggcagtggcaaaacctgttaaggaatggccaattggaacctcatctcctggtgcattctctactagccagtctttgtagccaaccatcctgtccatatattccaagacaaattcaaaggcaactttgtcttctgggcataacaaacagtacaatgctaaaggaggcagattgttaccataaatttcattccacttggcagcaaaatcagcatgctttggtggaggtaggtagtatgttgggttggacagcataactgtcactgcacttctgatagctctaaaaagatgcaaatggcttgcacgagacttttgtctcattgcttggatttctccagcatcaaaatataaacttggatgaagcatacttttcttcagcttttggttgggtctgaaatcttgcactttctgtgttttaaactgatctatatcatctgtgaaaactgcccattcggaataattgctcacagattcctcaaaagtagagaaagcaaacatcaataatgctaagaatagtaaatgtcctgtaaacattaacgccatgatccatgggggagctcctcccttaggcatacatgtcagatatgatgctcaatgtgtttcccatctggttagtataaaacatacagtaaaggccttgataagacaaagactgtaaatctgatatgctgtgaaatccagctgacattcagtacattttaagcaagtgcagttgccaaaaagagaaaacttaaattgtatatctctgtccctggcacagttttgcttccagtaaaactttgaataacgttaaaatctctaatttttccataatacacagggaagtgatacaggtaaaaaacactatgaatttagcatttacctcctttacttaaatctatttaacacaaagagttggaacacacattgtaaaaaaagagaaaaagcactccaaaattcaaattaagagtcatttctagcacagaaaaccatcactggtgataagctcaccacacatgtatgatgcatttgtgtatgtttgcccaaagaagatgatgaagtactgacattcttcgagtgagtggactcagttgtcattcctctcaactttttatacttcttgtcttgtgaatacgtttttctttcatttatgagagagaaacatcctcaacaagtgatcaaagtcttagttggtttttaaaaattcaaaattcttgccttcatttcaaatatttttcaggcttacttactcatcagcctattatgacaaagagaaatcatgttcacatcttcttttatcagcttcatgtgtacaaacataaaaatggaatatcttcagtcacctagatacttctcgtccgatcatgaagtaaccgccaacggggaaagaaaattcccctttcagcaacagtgaggtctctcttctgctcttttttcatgacacttttctcaggcagatcccgacgggggctcggcgccgcactgggccccaagggagacggaggtggagagttccagaaaactgctctgcacggcgggccaggctcccgcggggctccgcaagacccccgcgtcgtctcccgcgctacggcaggcgctgccccagctcggtctcctcagccgcgctcggtccccgcgacccgcacggcccggacacgcccgccctcaggaaacgccggacgcttgtgggggcaaccacggaccgcaggacagagacccgcgggcggcgggttctctcggtggcgccgtatccagagcagcgcccgcgtgcccaggcggtgatgtcgccgcggccgaggatcctctgt

SEQ ID NO: 11300 - RNA, 119 nt, Homo sapiens
  source 1..119: mol_type = other RNA
ctgaatagctgggactacaggtgcccgccaccacgcccggctaattttttgtattcttttagtagagatggggtttcaccgtgttagccacgacggtctcgatctcctgatttcgtgat

SEQ ID NO: 11301 - RNA, 1295 nt, Homo sapiens
  source 1..1295: mol_type = other RNA
ctgaatagctgggactacaggtgcccgccaccacgcccggctaattttttgtattttagtagagacagggtttcaccatgttgcccaggctggtctcaaactcctgagctcaggcaatccgcctgcctcaccctcccaaagtgctaggattacaggcatgagccaccactcccagccagtaatacttaaggctcatgctaggcttgaaaacaggtctactatactggcacagagaaataggtaagcatgagaccccggcactgggcacagctctctgctggggaaaccctgggagatggctcccctgcagggcggtttactcctggcctccagaagcttatctgttagtggaccgtgggcacacaagttttctttcccctttgtgtattcaccctcaaaagggcaaatttctacactataagttgttgctggactaacatcgaataataaagtacttctttagcaagattcaagttgaattcaatccttgtgaattctagaagcaattaacattatgagaatacagtagtccccctttatgtgaagtttcactttctgtggtttgttatccacagtcaacggcagctcaaaaatgggtgaacacacagcacaacaggatattttgagagagagagaaaacaaattcacataacttttaatagaacatatagttataactgttctattcttacttatttttgttaatttcttcctgtgcctaatttataaattaaactttatcacaggtatgtattacatacaggggaaaaacataatatatagagacttcagtactatcagtggtttcagacatccactggagatcttggaggtggataaggggggaccatggtgtttcaaaatcttgtttggagtttacaaagggaatgcttaatttctgatttatctaacaaaagatacctgtagacttacctgtcatacaaaataaccacactgaataatagcttgtcatagcaaatcttcccctccaactactcatacccctttctctctcttcaagtcctaaattcaagtaatacttcacttgacacttatttatctccaggattatcatataactaccattgacagttagatccacttttttgcaattgactgaacaacccaatcaatagcaacaaggacactctgctttcacaagatgacagctgctccagctgctggctccctggggctgatgttggggaatcaggccagcacaacatgacacattcacagggacacggacaccaggtacaacactacatctacatgggtcattagcttgactatag

SEQ ID NO: 11302 - RNA, 1941 nt, Homo sapiens
  source 1..1941: mol_type = other RNA
ctgaatagctgggactacaggtgcccgccaccacgcccggctaattttttgtatttttagtagagacagggtttcactgtgttatccaggatggtcttgatctcctcaccttgtgatccgcccaccttggcctcccaaaatgctgggattacaggcgtgagccaccacgcccggcccacaagtgggtttttaaaaggaaagaagaggcagttcctgagttatttaccaataatttacattaacataacataagctgttgattggctatccattattaagctataggatatgggttataatgtctggtgcagcaccagtaggctaattttcagctacttgtggcaatagtaagcagtataaaaagatgagtacatgcctcaaaagggggtgtgtgtaggacaggattgccgtctcattttaatacctctctggatctgataattggaaaggacttgcattcttcagataaaagttctttttctcatttcttccttttgatcaaaaatctttccttttgaaagcactgatgatcaaaatctgagtgtcaaggtatccctcattgccagaaaggctcatgcccaggtagtcctaccagtcattgatttatagctgccatcacttgtggaatcacctcttcagtgtaccatgaatttagttttctcagaagaaataaaacaatgagagatacacagcggaaatattttgaggttcccaggcctgtcagaaagtgacattctttacttaacacaggacagaaatcttgaaagggaactacgtagacaagggaccaggccagtctttccaagaggctttctaattgcctctatagagtcaacctccattcttcaaagcagtctggtcatatctgaaaatatgtcattccagtcaaatccttagtaaaataacaagtgtctccaattatatcctgaaagttgttacttagtccaatgatatgatctccaaagttatcagaaacctgtattcaagagtacttgtcagggtcctattctatgaatttcctcttgaatgaaggtgactttttctttcaggatttcttttagaagtttttaggtgccagtggaagtcagtctcttatttacatgtctggttctaaaaccagctctttccaatggtgtgcacaaataaattactttaggtatatcaaaagatccccatttttggtcattgttgcctatgatcattccaggttagatgggtctactttcccagatactacaagacagtaccccataaatcatatatgtagttccagcaggtatttctaaaaagagtgttcaggttttgaacactcttattattgatttctcataactcaggaacttttcaaaagtgaccaaagccaggaatgtgtttaggatcaaagtgtggcatgttttggactgtctctaattgtcagatggcagcagagtcctcaaggatgaggacaattggattgtctgtaattgtcagatggcagcggagtcctcaaggtatgggggaccagaccctcgtattacgtccacctgatgagacttctgaaggaagagagttcacactggtaccaagcgctgctttcagagagaaacaccaccagctggttggggggagtcactgtgaatcctgctgacttactccagatgttttacttggtcatttcctgagaaactctttgcttgaatttttccactcttcaggtgaagatgatgacactgtccaggctttcaggagtccaacctcttagacaataagcgacatactctttggtaactgcagtggctctgcttgtaagaaaagtcctttgcgccattcccctccaagccccagggaagggcctggaaagcgcttacacctcagacccagtgtcggtcagccgtcaaggagcgagcgacgtgggaaaccctgagataggacattggcccggcgctgggctcgggtaacgat

SEQ ID NO: 11303 - RNA, 3957 nt, Homo sapiens
  source 1..3957: mol_type = other RNA
ctgaatagctgggactacaggtgcccgccaccacgcccggctaattttttgtatttttagtagagacggggtttcacgtgttagccaggatggtctcgatctcctgacctcatgatccacccgcctcggcctcccaaagtgctgggattacaggcgtgagccactgcgcccggcctcaccgtgcatgttttaaacacatacccatcaacgacaagattggggaagtgaatggcttggaggcatttgcatagaagtggaagcactaggtgggcggacataaagacgacaatggcagttctcgatattcacgatcacggctttgaagtcccggtcaacctgcccctctctgtccccggcattcattgacacgggctttccctggcctgggatcccatcccaacacacacgacagaaaacagtgcaaaataataacacaaatgccaaatgtacacagtgtacaactctgaactgagaaagtgcaaggagaccacgggaatggaagtgggtaggggtcgggaggatgggcaccaggctggtgtcctgacagccacacctgggtgcaggccacgtgtcctcacggccaaggtaaccgggtgtctcaggcacttaataaatattaagggtgaccagtgactcaggctctgcctctgggaagtggcatcatttggtgaatgagtttggtctcggtgccaccacggattcagccagatcatttccgacgccatgaatccctttcctggcttaaggaaggtacaaacccacctcgaaagacactgggtgggtcatgattcgggggtgacagggcaaaggctaacctggctgtctagcaaggcttgcatagaagaggtaaacacgttgactcctgagtttaggggtttggcttagagattggtggatgaggcagggccagggggtcccgttggtgccatctgctgttgtgtgttgaaagccacttgcttctctgggcctgacatcccctcccctttcatcttccatgtttgaggattgtgtcacggtggagagaaactcaaaacttcctggagagaaatggaggtgtcatcctggtccccccgggcctgtttctcttatccttcacgaggaaaggaagaaaccaaaatcccaacccaagccattgcatgggcactgtccgaagcctgttctgcctcccagatgaataaatatataaaacaaagctctggcaggcaatgctttggtcttctctgtctttgaataaaacaaggccggcgaggtctcaggaagggttctgggcagggacgggactccaggcagatgttcacgccacgtcatcctccagactgaccatcgaggggtagctgtagccgtcctggttgtggcaaatgtggacctcatcctctgtggtcttctgatagacggggttgtcaaagttgatgctgttgatgttcttaagccgccagttcttccatagaaggaagacccccaggcaaaggaagacgaggagcacgatggggaggacaatggacagagccctcacgctactgggcttcttctcatttcctctgccagcaacgtcgcccagagcttggtgagacattgtcactatctccaccgtggtgagcccaggggtggccccaggcagccgggaggtgtcgggaacaggtcgggtggttgtgtgctgtgtccttacggctgtggagctgacctttagcctgacggtggatgtctcctgggtggccactgcagcctcagcctctgtgaggcagctcctcatgtccctggccagcagcatgccgtccgggcaggcgcaggtaaacttgggcgagtgggggttgatctgcggggcagggaggcacagatactggcagccgccattgctcagggtggtcctctcacaccagttcactcctcttggctgggtgaggttgtggaagagaaccatatcctctggggacagtaggttttcagccaacaagttgacatcggaacctgtgaggcggttggcactgaaaatggcttcgttgatgatatctgtccaaaatactttgtcctcaaagacggccaaggagaaggggtgggccagcctcttttcatcctccaagatggtcttccggttgcccccgttgacatcgatgcttgagatggagtgaagtttggagtcaacccagtagaggcggccactgaggagatctagggtgatgccattgggccactgaatgttttcagtcaccagcgagtagatgtccacaccattcaggccccctttcttgatcttggcgggagttccccagtcagtccagtacatgaagccatgaacaggatccaccacgatggcccttggcttggagccgttctccctgaataacgttttcctcttcacgcccttggtatccgcaacagagacagtgcccaggacagagtcggtccagtagatgttgctgtggatccagtccacagccagcccgtcgggggcctggatgtctctgctgatgacggtgtcataggaagagacgccgtgggctctgtcaagctgggtgctgcagatcattctctgggacaggtcagaccagtagattctattgctggccacctccgtgtccagagcgaccacgttcctcaggttggggatgaggctggtgtactcgctccggtccagcgtcatcttcctgacctcgtgccggttggtgaagaagaggtaggcgatggagcccacagccttgcaggccttcgtgtgggggtccagctggaagccttcctcacactggcacttgtagccaccctccaggttcacgcagagctggctgcaggtgtcgggatcctgacactcatcgatatcttcgcatcttcgctgggccaccagctggaagccgtcggggcacaggcactcgtagccgatcttaaggtcattgcagacgtgggaacagccgccgttgttgtccaagcattcgttggtcccgcactctttgatgggttcatctgaccagtcccggcagtctctagccatgttgcagactttgtccagggtgatgcattcgccgctgtgacacttgaacttgttgggtccctcgcagagtgtcacattaacgcagccaacttcatcgctcatgtccttgcagtcatattcccggtcacactgccggctgccatggatgcagtttccatcagagcactggaattcgtcagggcgacaggtggccacagcgcagttttcctcgtcagatttgtccttgcagtcggggccaccatcacagcgccagctggagtggatgcactcgccacttaggcagtggaactcgaaggccgagcaggggctactgtccccttggaacacgtaaagacccctacagcgctgcggccactcatccgagccatcttcgcagtcggggtcgttgtcgcaggcccacagctgggggatgcaggtggagctgttgcactggaagctggcgggaccacaggtgagcaccgggcaggaggcctcgtctgagccgtccaagcagtcccggtctgagtcacagacgaactgccgagagatgcacttcccatcgtggcagcgaaactcgtcctgggagcacgtcttggggggacagccttgctcgtctgagccgttgtcgcagtccacttggccatcgcacctccagaactgaggaatgcagcggttgacacggcccccacagctgaagtccccggatttgcaggtgacagacaagcacgtctcctgggactcatcagagccatcctggcactcagcgctgccatcgcagacccacttgtaggagatgcatttcccgtcttggcactggaactcgtttctttcgcatctgtcgcccactgcagtccccgccgcggcgaggagcaaggcgacggtccagcgcaatttccagccccagggccccatgctcgcagcctctgccaggcagtgtcccgacccggatcacgacctgctgtgtcctagctggaaaccctggcttcccgcgattgcac

SEQ ID NO: 11304 - RNA, 4211 nt, Homo sapiens
  source 1..4211: mol_type = other RNA
ctgaatagctgggactacaggtgcccgccaccacgcccggctaattttttgtatttttagtagagacggggtttcacgtgttagccaggatggtctcgatctcctgacctcatgatccacccgcctcggcctcccaaagtgctgggattacaggcgtgagccactgcgcccggcctcaccgtgcatgttttaaacacatacccatcaacgacaagattggggaagtgaatggcttggaggcatttgcatagaagtggaagcactaggtgggcggacataaagacgacaatggcagttctcgatattcacgatcacggctttgaagtcccggtcaacctgcccctctctgtccccggcattcattgacacgggctttccctggcctgggatcccatcccaacacacacgacagaaaacagtgcaaaataataacacaaatgccaaatgtacacagtgtacaactctgaactgagaaagtgcaaggagaccacgggaatggaagtgggtaggggtcgggaggatgggcaccaggctggtgtcctgacagccacacctgggtgcaggccacgtgtcctcacggccaaggtaaccgggtgtctcaggcacttaataaatattaagggtgaccagtgactcaggctctgcctctgggaagtggcatcatttggtgaatgagtttggtctcggtgccaccacggattcagccagatcatttccgacgccatgaatccctttcctggcttaaggaaggtacaaacccacctcgaaagacactgggtgggtcatgattcgggggtgacagggcaaaggctaacctggctgtctagcaaggcttgcatagaagaggtaaacacgttgactcctgagtttaggggtttggcttagagattggtggatgaggcagggccagggggtcccgttggtgccatctgctgttgtgtgttgaaagccacttgcttctctgggcctgacatcccctcccctttcatcttccatgtttgaggattgtgtcacggtggagagaaactcaaaacttcctggagagaaatggaggtgtcatcctggtccccccgggcctgtttctcttatccttcacgaggaaaggaagaaaccaaaatcccaacccaagccattgcatgggcactgtccgaagcctgttctgcctcccagatgaataaatatataaaacaaagctctggcaggcaatgctttggtcttctctgtctttgaataaaacaaggccggcgaggtctcaggaagggttctgggcagggacgggactccaggcagatgttcacgccacgtcatcctccagactgaccatctgtctcgaggggtagctgtagccgtcctggttgtggcaaatgtggacctcatcctctgtggtcttctgatagacggggttgtcaaagttgatgctgttgatgttcttaagccgccagttcttccatagaaggaagacccccaggcaaaggaagacgaggagcacgatggggaggacaatggacagagccctcacgctactgggcttcttctcatttcctctgccagcaacgtcgcccagagcttggtgagacattgtcactatctccaccgtggtgagcccaggggtggccccaggcagccgggaggtgtcgggaacaggtcgggtggttgtgtgctgtgtccttacggctgtggagctgacctttagcctgacggtggatgtctcctgggtggccactgcagcctcagcctctcttcagggggccgggaaagaggaaaccaggcatcaaaggggaactgggtaaatgtcaagcccggtgctgatgtgtccatccaagaaaagtatggttatcccgactcatgagtccttacaacgaccttgaggtacccatttgacagatgagcagagagaggctcaggagggggcagttggaggacacaggacgcagaaacaaggcgtgtgccacacctgtgaggcagctcctcatgtccctggccagcagcatgccgtccgggcaggcgcaggtaaacttgggcgagtgggggttgatctgcggggcagggaggcacagatactggcagccgccattgctcagggtggtcctctcacaccagttcactcctcttggctgggtgaggttgtggaagagaaccatatcctctggggacagtaggttttcagccaacaagttgacatcggaacctgtgaggcggttggcactgaaaatggcttcgttgatgatatctgtccaaaatactttgtcctcaaagacggccaaggagaaggggtgggccagcctcttttcatcctccaagatggtcttccggttgcccccgttgacatcgatgcttgagatggagtgaagtttggagtcaacccagtagaggcggccactgaggagatctagggtgatgccattgggccactgaatgttttcagtcaccagcgagtagatgtccacaccattcaggccccctttcttgatcttggcgggagttccccagtcagtccagtacatgaagccatgaacaggatccaccacgatggcccttggcttggagccgttctccctgaataacgttttcctcttcacgcccttggtatccgcaacagagacagtgcccaggacagagtcggtccagtagatgttgctgtggatccagtccacagccagcccgtcgggggcctggatgtctctgctgatgacggtgtcataggaagagacgccgtgggctctgtcaagctgggtgctgcagatcattctctgggacaggtcagaccagtagattctattgctggccacctccgtgtccagagcgaccacgttcctcaggttggggatgaggctggtgtactcgctccggtccagcgtcatcttcctgacctcgtgccggttggtgaagaagaggtaggcgatggagcccacagccttgcaggccttcgtgtgggggtccagctggaagccttcctcacactggcacttgtagccaccctccaggttcacgcagagctggctgcaggtgtcgggatcctgacactcatcgatatcttcgcatcttcgctgggccaccagctggaagccgtcggggcacaggcactcgtagccgatcttaaggtcattgcagacgtgggaacagccgccgttgttgtccaagcattcgttggtcccgcactctttgatgggttcatctgaccagtcccggcagtctctagccatgttgcagactttgtccagggtgatgcattcgccgctgtgacacttgaacttgttgggtccctcgcagagtgtcacattaacgcagccaacttcatcgctcatgtccttgcagtcatattcccggtcacactgccggctgccatggatgcagtttccatcagagcactggaattcgtcagggcgacaggtggccacagcgcagttttcctcgtcagatttgtccttgcagtcggggccaccatcacagcgccagctggagtggatgcactcgccacttaggcagtggaactcgaaggccgagcaggggctactgtccccttggaacacgtaaagacccctacagcgctgcggccactcatccgagccatcttcgcagtcggggtcgttgtcgcaggcccacagctgggggatgcaggtggagctgttgcactggaagctggcgggaccacaggtgagcaccgggcaggaggcctcgtctgagccgtccaagcagtcccggtctgagtcacagacgaactgccgagagatgcacttcccatcgtggcagcgaaactcgtcctgggagcacgtcttggggggacagccttgctcgtctgagccgttgtcgcagtccacttggccatcgcacctccagaactgaggaatgcagcggttgacacggcccccacagctgaagtccccggatttgcaggtgacagacaagcacgtctcctgggactcatcagagccatcctggcactcagcgctgccatcgcagacccacttgtaggagatgcatttcccgtcttggcactggaactcgtttctttcgcatctgtcgcccactgcagtccccgccgcggcgaggagcaaggcgacggtccagcgcaatttccagccccagggccccatgctcgcagcctctgccaggcagtgtcccgacccggatcacgacctgctgtgtcctagctggaaaccctggcttcccgcgattgcactcggggcccacgtcatttacagcatttcaat

SEQ ID NO: 11305 - RNA, 3429 nt, Homo sapiens
  source 1..3429: mol_type = other RNA
ctgaatagctgggactacaggtgcccgccaccacgcccggctaattttttgtatttttagtagagacggggtttcacgtgttagccaggatggtctcgatctcctgacctcatgatccacccgcctcggcctcccaaagtgctgggattacaggcgtgagccactgcgcccggcctcaccgtgcatgttttaaacacatacccatcaacgacaagattggggaagtgaatggcttggaggcatttgcatagaagtggaagcactaggtgggcggacataaagacgacaatggcagttctcgatattcacgatcacggctttgaagtcccggtcaacctgcccctctctgtccccggcattcattgacacgggctttccctggcctgggatcccatcccaacacacacgacagaaaacagtgcaaaataataacacaaatgccaaatgtacacagtgtacaactctgaactgagaaagtgcaaggagaccacgggaatggaagtgggtaggggtcgggaggatgggcaccaggctggtgtcctgacagccacacctgggtgcaggccacgtgtcctcacggccaaggtaaccgggtgtctcaggcacttaataaatattaagggtgaccagtgactcaggctctgcctctgggaagtggcatcatttggtgaatgagtttggtctcggtgccaccacggattcagccagatcatttccgacgccatgaatccctttcctggcttaaggaaggtacaaacccacctcgaaagacactgggtgggtcatgattcgggggtgacagggcaaaggctaacctggctgtctagcaaggcttgcatagaagaggtaaacacgttgactcctgagtttaggggtttggcttagagattggtggatgaggcagggccagggggtcccgttggtgccatctgctgttgtgtgttgaaagccacttgcttctctgggcctgacatcccctcccctttcatcttccatgtttgaggattgtgtcacggtggagagaaactcaaaacttcctggagagaaatggaggtgtcatcctggtccccccgggcctgtttctcttatccttcacgaggaaaggaagaaaccaaaatcccaacccaagccattgcatgggcactgtccgaagcctgttctgcctcccagatgaataaatatataaaacaaagctctggcaggcaatgctttggtcttctctgtctttgaataaaacaaggccggcgaggtctcaggaagggttctgggcagggacgggactccaggcagatgttcacgccacgtcatcctccagactgaccatctgtctcgaggggtagctgtagccgtcctggttgtggcaaatgtggacctcatcctctgtggtcttctgatagacggggttgtcaaagttgatgctgttgatgttcttaagccgccagttcttccatagaaggaagacccccaggcaaaggaagacgaggagcacgatggggaggacaatggacagagccctcacgctactgggcttcttctcatttcctctgccagcaacgtcgcccagagcttggtgagacattgtcactatctccaccgtggtgagcccaggggtggccccaggcagccgggaggtgtcgggaacaggtcgggtggttgtgtgctgtgtccttacggctgtggagctgacctttagcctgacggtggatgtctcctgggtggccactgcagcctcagcctctcttggctgggtgaggttgtggaagagaaccatatcctctggggacagtaggttttcagccaacaagttgacatcggaacctgtgaggcggttggcactgaaaatggcttcgttgatgatatctgtccaaaatactttgtcctcaaagacggccaaggagaaggggtgggccagcctcttttcatcctccaagatggtcttccggttgcccccgttgacatcgatgcttgagatggagtgaagtttggagtcaacccagtagaggcggccactgaggagatctagggtgatgccattgggccactgaatgttttcagtcaccagcgagtagatgtccacaccattcaggccccctttcttgatcttggcgggagttccccagtcagtccagtacatgaagccatgaacaggatccaccacgatggcccttggcttggagccgttctccctgaataacgttttcctcttcacgcccttggtatccgcaacagagacagtgcccaggacagagtcggtccagtagatgttgctgtggatccagtccacagccagcccgtcgggggcctggatgtctctgctgatgacggtgtcataggaagagacgccgtgggctctgtcaagctgggtgctgcagatcattctctgggacaggtcagaccagtagattctattgctggccacctccgtgtccagagcgaccacgttcctcaggttggggatgaggctggtgtactcgctccggtccagcgtcatcttcctgacctcgtgccggttggtgaagaagaggtaggcgatggagcccacagccttgcaggccttcgtgtgggggtccagctggaagccttcctcacactggcacttgtagccaccctccaggttcacgcagagctggctgcaggtgtcgggatcctgacactcatcgatatcttcgcatcttcgctgggccaccagctggaagccgtcggggcacaggcactcgtagccgatcttaaggtcattgcagacgtgggaacagccgccgttgttgtccaagcattcgttggtcccgcactctttgatgggttcatctgaccagtcccggcagtctctagccatgttgcagactttgtccagggtgatgcattcgccgctgtgacacttgaacttgttgggtccctcgcagagtgtcacattaacgcagccaacttcatcgctcatgtccttgcagtcatattcccggtcacactgccggctgccatggatgcagtttccatcagagcactggaattcgtcagggcgacaggtggccacaggacagccttgctcgtctgagccgttgtcgcagtccacttggccatcgcacctccagaactgaggaatgcagcggttgacacggcccccacagctgaagtccccggatttgcaggtgacagacaagcacgtctcctgggactcatcagagccatcctggcactcagcgctgccatcgcagacccacttgtaggagatgcatttcccgtcttggcactggaactcgtttctttcgcatctgtcgcccactgcagtccccgccgcggcgaggagcaaggcgacggtccagcgcaatttccagccccagggccccatgctcgcagcctctgccaggcagtgtcccgacccggatcacgacctgctgtgtcctagctggaaaccctggcttcccgcgattgcac

SEQ ID NO: 11306 - RNA, 3854 nt, Homo sapiens
  source 1..3854: mol_type = other RNA
ctgaatagctgggactacaggtgcccgccaccacgcccggctaattttttgtatttttagtagagacggggtttcacgtgttagccaggatggtctcgatctcctgacctcatgatccacccgcctcggcctcccaaagtgctgggattacaggcgtgagccactgcgcccggcctcaccgtgcatgttttaaacacatacccatcaacgacaagattggggaagtgaatggcttggaggcatttgcatagaagtggaagcactaggtgggcggacataaagacgacaatggcagttctcgatattcacgatcacggctttgaagtcccggtcaacctgcccctctctgtccccggcattcattgacacgggctttccctggcctgggatcccatcccaacacacacgacagaaaacagtgcaaaataataacacaaatgccaaatgtacacagtgtacaactctgaactgagaaagtgcaaggagaccacgggaatggaagtgggtaggggtcgggaggatgggcaccaggctggtgtcctgacagccacacctgggtgcaggccacgtgtcctcacggccaaggtaaccgggtgtctcaggcacttaataaatattaagggtgaccagtgactcaggctctgcctctgggaagtggcatcatttggtgaatgagtttggtctcggtgccaccacggattcagccagatcatttccgacgccatgaatccctttcctggcttaaggaaggtacaaacccacctcgaaagacactgggtgggtcatgattcgggggtgacagggcaaaggctaacctggctgtctagcaaggcttgcatagaagaggtaaacacgttgactcctgagtttaggggtttggcttagagattggtggatgaggcagggccagggggtcccgttggtgccatctgctgttgtgtgttgaaagccacttgcttctctgggcctgacatcccctcccctttcatcttccatgtttgaggattgtgtcacggtggagagaaactcaaaacttcctggagagaaatggaggtgtcatcctggtccccccgggcctgtttctcttatccttcacgaggaaaggaagaaaccaaaatcccaacccaagccattgcatgggcactgtccgaagcctgttctgcctcccagatgaataaatatataaaacaaagctctggcaggcaatgctttggtcttctctgtctttgaataaaacaaggccggcgaggtctcaggaagggttctgggcagggacgggactccaggcagatgttcacgccacgtcatcctccagactgaccatctgtctcgaggggtagctgtagccgtcctggttgtggcaaatgtggacctcatcctctgtggtcttctgatagacggggttgtcaaagttgatgctgttgatgttcttaagccgccagttcttccatagaaggaagacccccaggcaaaggaagacgaggagcacgatggggaggacaatggacagagccctcacgctactgggcttcttctcatttcctctgccagcaacgtcgcccagagcttggtgagacattgtcactatctccaccgtggtgagcccaggggtggccccaggcagccgggaggtgtcgggaacaggtcgggtggttgtgtgctgtgtccttacggctgtggagctgacctttagcctgacggtggatgtctcctgggtggccactgcagcctcagcctctgtgaggcagctcctcatgtccctggccagcagcatgccgtccgggcaggcgcaggtaaacttgggcgagtgggggttgatctgcggggcagggaggcacagatactggcagccgccattgctcagggtggtcctctcacaccagttcactcctcttggctgggtgaggttgtggaagagaaccatatcctctggggacagtaggttttcagccaacaagttgacatcggaacctgtgaggcggttggcactgaaaatggcttcgttgatgatatctgtccaaaatactttgtcctagggtgatgccattgggccactgaatgttttcagtcaccagcgagtagatgtccacaccattcaggccccctttcttgatcttggcgggagttccccagtcagtccagtacatgaagccatgaacaggatccaccacgatggcccttggcttggagccgttctccctgaataacgttttcctcttcacgcccttggtatccgcaacagagacagtgcccaggacagagtcggtccagtagatgttgctgtggatccagtccacagccagcccgtcgggggcctggatgtctctgctgatgacggtgtcataggaagagacgccgtgggctctgtcaagctgggtgctgcagatcattctctgggacaggtcagaccagtagattctattgctggccacctccgtgtccagagcgaccacgttcctcaggttggggatgaggctggtgtactcgctccggtccagcgtcatcttcctgacctcgtgccggttggtgaagaagaggtaggcgatggagcccacagccttgcaggccttcgtgtgggggtccagctggaagccttcctcacactggcacttgtagccaccctccaggttcacgcagagctggctgcaggtgtcgggatcctgacactcatcgatatcttcgcatcttcgctgggccaccagctggaagccgtcggggcacaggcactcgtagccgatcttaaggtcattgcagacgtgggaacagccgccgttgttgtccaagcattcgttggtcccgcactctttgatgggttcatctgaccagtcccggcagtctctagccatgttgcagactttgtccagggtgatgcattcgccgctgtgacacttgaacttgttgggtccctcgcagagtgtcacattaacgcagccaacttcatcgctcatgtccttgcagtcatattcccggtcacactgccggctgccatggatgcagtttccatcagagcactggaattcgtcagggcgacaggtggccacagcgcagttttcctcgtcagatttgtccttgcagtcggggccaccatcacagcgccagctggagtggatgcactcgccacttaggcagtggaactcgaaggccgagcaggggctactgtccccttggaacacgtaaagacccctacagcgctgcggccactcatccgagccatcttcgcagtcggggtcgttgtcgcaggcccacagctgggggatgcaggtggagctgttgcactggaagctggcgggaccacaggtgagcaccgggcaggaggcctcgtctgagccgtccaagcagtcccggtctgagtcacagacgaactgccgagagatgcacttcccatcgtggcagcgaaactcgtcctgggagcacgtcttggggggacagccttgctcgtctgagccgttgtcgcagtccacttggccatcgcacctccagaactgaggaatgcagcggttgacacggcccccacagctgaagtccccggatttgcaggtgacagacaagcacgtctcctgggactcatcagagccatcctggcactcagcgctgccatcgcagacccacttgtaggagatgcatttcccgtcttggcactggaactcgtttctttcgcatctgtcgcccactgcagtccccgccgcggcgaggagcaaggcgacggtccagcgcaatttccagccccagggccccatgctcgcagcctctgccaggcagtgtcccgacccggatcacgacctgctgtgtcctagctggaaaccctggcttcccgcgattgcactcggggcccacgtcatttacagcatttcaat

SEQ ID NO: 11307 - RNA, 3840 nt, Homo sapiens
  source 1..3840: mol_type = other RNA
ctgaatagctgggactacaggtgcccgccaccacgcccggctaattttttgtatttttagtagagacggggtttcacgtgttagccaggatggtctcgatctcctgacctcatgatccacccgcctcggcctcccaaagtgctgggattacaggcgtgagccactgcgcccggcctcaccgtgcatgttttaaacacatacccatcaacgacaagattggggaagtgaatggcttggaggcatttgcatagaagtggaagcactaggtgggcggacataaagacgacaatggcagttctcgatattcacgatcacggctttgaagtcccggtcaacctgcccctctctgtccccggcattcattgacacgggctttccctggcctgggatcccatcccaacacacacgacagaaaacagtgcaaaataataacacaaatgccaaatgtacacagtgtacaactctgaactgagaaagtgcaaggagaccacgggaatggaagtgggtaggggtcgggaggatgggcaccaggctggtgtcctgacagccacacctgggtgcaggccacgtgtcctcacggccaaggtaaccgggtgtctcaggcacttaataaatattaagggtgaccagtgactcaggctctgcctctgggaagtggcatcatttggtgaatgagtttggtctcggtgccaccacggattcagccagatcatttccgacgccatgaatccctttcctggcttaaggaaggtacaaacccacctcgaaagacactgggtgggtcatgattcgggggtgacagggcaaaggctaacctggctgtctagcaaggcttgcatagaagaggtaaacacgttgactcctgagtttaggggtttggcttagagattggtggatgaggcagggccagggggtcccgttggtgccatctgctgttgtgtgttgaaagccacttgcttctctgggcctgacatcccctcccctttcatcttccatgtttgaggattgtgtcacggtggagagaaactcaaaacttcctggagagaaatggaggtgtcatcctggtccccccgggcctgtttctcttatccttcacgaggaaaggaagaaaccaaaatcccaacccaagccattgcatgggcactgtccgaagcctgttctgcctcccagatgaataaatatataaaacaaagctctggcaggcaatgctttggtcttctctgtctttgaataaaacaaggccggcgaggtctcaggaagggttctgggcagggacgggactccaggcagatgttcacgccacgtcatcctccagactgaccatctgtctcgaggggtagctgtagccgtcctggttgtggcaaatgtggacctcatcctctgtggtcttctgatagacggggttgtcaaagttgatgctgttgatgttcttaagccgccagttcttccatagaaggaagacccccaggcaaaggaagacgaggagcacgatggggaggacaatggacagagccctcacgctactgggcttcttctcatttcctctgccagcaacgtcgcccagagcttggtgagacattgtcactatctccaccgtggtgagcccaggggtggccccaggcagccgggaggtgtcgggaacaggtcgggtggttgtgtgctgtgtccttacggctgtggagctgacctttagcctgacggtggatgtctcctgggtggccactgcagcctcagcctctgtgaggcagctcctcatgtccctggccagcagcatgccgtccgggcaggcgcaggtaaacttgggcgagtgggggttgatctgcggggcagggaggcacagatactggcagccgccattgctcagggtggtcctctcacaccagttcactcctcttggctgggtgaggttgtggaagagaaccatatcctctggggacagtaggttttcagccaacaagttgacatcggaacctgtgaggcggttggcactgaaaatggcttcgttgatgatatctgtccaaaatactttgtcctcaaagacggccaaggagaaggggtgggccagcctcttttcatcctccaagatggtcttccggttgcccccgttgacatcgatgcttgagatggagtgaagtttggagtcaacccagtagaggcggccactgaggagatctagggtgatgccattgggccactgaatgttttcagtcaccagcgagtagatgtccacaccattcaggccccctttcttgatcttggcgggagttccccagtcagtccagtacatgaagccatgaacaggatccaccacgatggcccttggcttggagccgttctccctgaataacgttttcctcttcacgcccttggtatccgcaacagagacagtgcccaggacagagtcggtccagtagatgttgctgtggatccagtccacagccagcccgtcgggggcctggatgtctctgctgatgacggtgtcataggaagagacgccgtgggctctgtcaagctgggtgctgcagatcattctctgggacaggtcagaccagtagattctattgctggccacctccgtgtccagagcgaccacgttcctcaggttggggatgaggctggtgtactcgctccggtccagcgtcatcttcctgacctcgtgccggttggtgaagaagaggtaggcgatggagcccacagccttgcaggccttcgtgtgggggtccagctggaagccttcctcacactggcacttgtagccaccctccaggttcacgcagagctggctgcaggtgtcgggatcctgacactcatcgatatcttcgcatcttcgctgggccaccagctggaagccgtcggggcacaggcactcgtagccgatcttaaggtcattgcagacgtgggaacagccgccgttgttgtccaagcattcgttggtcccgcactctttgatgggttcatctgaccagtcccggcagtctctagccatgttgcagactttgtccagggtgatgcattcgccgctgtgacacttgaacttgttgggtccctcgcagagtgtcacattaacgcagccaacttcatcgctcatgtccttgcagtcatattcccggtcacactgccggctgccatggatgcagtttccatcagagcactggaattcgtcagggcgacaggtggccacagcgcagttttcctcgtcagatttgtccttgcagtcggggccaccatcacagcgccagctggagtggatgcactcgccacttaggcagtggaactcgaaggccgagcaggggctactgtccccttggaacacgtaaagacccctacagcgctgcggccactcatccgagccatcttcgcagtcggggtcgttgtcgcaggcccacagctgggggatgcaggtggagctgttgcactggaagctggcgggaccacaggtgagcaccgggcaggaggcctcgtctgagccgtccaagcagtcccggtctgagtcacagacgaactgccgagagatgcacttcccatcgtggcagcgaaactcgtcctgggagcacgtcttgggggagcacgtctcctgggactcatcagagccatcctggcactcagcgctgccatcgcagacccacttgtaggagatgcatttcccgtcttggcactggaactcgtttctttcgcatctgtcgcccactgcagtccccgccgcggcgaggagcaaggcgacggtccagcgcaatttccagccccagggccccatgctcgcagcctctgccaggcagtgtcccgacccggatcacgacctgctgtgtcctagctggaaaccctggcttcccgcgattgcac

SEQ ID NO: 11308 - RNA, 3963 nt, Homo sapiens
  source 1..3963: mol_type = other RNA
ctgaatagctgggactacaggtgcccgccaccacgcccggctaattttttgtatttttagtagagacggggtttcacgtgttagccaggatggtctcgatctcctgacctcatgatccacccgcctcggcctcccaaagtgctgggattacaggcgtgagccactgcgcccggcctcaccgtgcatgttttaaacacatacccatcaacgacaagattggggaagtgaatggcttggaggcatttgcatagaagtggaagcactaggtgggcggacataaagacgacaatggcagttctcgatattcacgatcacggctttgaagtcccggtcaacctgcccctctctgtccccggcattcattgacacgggctttccctggcctgggatcccatcccaacacacacgacagaaaacagtgcaaaataataacacaaatgccaaatgtacacagtgtacaactctgaactgagaaagtgcaaggagaccacgggaatggaagtgggtaggggtcgggaggatgggcaccaggctggtgtcctgacagccacacctgggtgcaggccacgtgtcctcacggccaaggtaaccgggtgtctcaggcacttaataaatattaagggtgaccagtgactcaggctctgcctctgggaagtggcatcatttggtgaatgagtttggtctcggtgccaccacggattcagccagatcatttccgacgccatgaatccctttcctggcttaaggaaggtacaaacccacctcgaaagacactgggtgggtcatgattcgggggtgacagggcaaaggctaacctggctgtctagcaaggcttgcatagaagaggtaaacacgttgactcctgagtttaggggtttggcttagagattggtggatgaggcagggccagggggtcccgttggtgccatctgctgttgtgtgttgaaagccacttgcttctctgggcctgacatcccctcccctttcatcttccatgtttgaggattgtgtcacggtggagagaaactcaaaacttcctggagagaaatggaggtgtcatcctggtccccccgggcctgtttctcttatccttcacgaggaaaggaagaaaccaaaatcccaacccaagccattgcatgggcactgtccgaagcctgttctgcctcccagatgaataaatatataaaacaaagctctggcaggcaatgctttggtcttctctgtctttgaataaaacaaggccggcgaggtctcaggaagggttctgggcagggacgggactccaggcagatgttcacgccacgtcatcctccagactgaccatctgtctcgaggggtagctgtagccgtcctggttgtggcaaatgtggacctcatcctctgtggtcttctgatagacggggttgtcaaagttgatgctgttgatgttcttaagccgccagttcttccatagaaggaagacccccaggcaaaggaagacgaggagcacgatggggaggacaatggacagagccctcacgctactgggcttcttctcatttcctctgccagcaacgtcgcccagagcttggtgagacattgtcactatctccaccgtggtgagcccaggggtggccccaggcagccgggaggtgtcgggaacaggtcgggtggttgtgtgctgtgtccttacggctgtggagctgacctttagcctgacggtggatgtctcctgggtggccactgcagcctcagcctctgtgaggcagctcctcatgtccctggccagcagcatgccgtccgggcaggcgcaggtaaacttgggcgagtgggggttgatctgcggggcagggaggcacagatactggcagccgccattgctcagggtggtcctctcacaccagttcactcctcttggctgggtgaggttgtggaagagaaccatatcctctggggacagtaggttttcagccaacaagttgacatcggaacctgtgaggcggttggcactgaaaatggcttcgttgatgatatctgtccaaaatactttgtcctcaaagacggccaaggagaaggggtgggccagcctcttttcatcctccaagatggtcttccggttgcccccgttgacatcgatgcttgagatggagtgaagtttggagtcaacccagtagaggcggccactgaggagatctagggtgatgccattgggccactgaatgttttcagtcaccagcgagtagatgtccacaccattcaggccccctttcttgatcttggcgggagttccccagtcagtccagtacatgaagccatgaacaggatccaccacgatggcccttggcttggagccgttctccctgaataacgttttcctcttcacgcccttggtatccgcaacagagacagtgcccaggacagagtcggtccagtagatgttgctgtggatccagtccacagccagcccgtcgggggcctggatgtctctgctgatgacggtgtcataggaagagacgccgtgggctctgtcaagctgggtgctgcagatcattctctgggacaggtcagaccagtagattctattgctggccacctccgtgtccagagcgaccacgttcctcaggttggggatgaggctggtgtactcgctccggtccagcgtcatcttcctgacctcgtgccggttggtgaagaagaggtaggcgatggagcccacagccttgcaggccttcgtgtgggggtccagctggaagccttcctcacactggcacttgtagccaccctccaggttcacgcagagctggctgcaggtgtcgggatcctgacactcatcgatatcttcgcatcttcgctgggccaccagctggaagccgtcggggcacaggcactcgtagccgatcttaaggtcattgcagacgtgggaacagccgccgttgttgtccaagcattcgttggtcccgcactctttgatgggttcatctgaccagtcccggcagtctctagccatgttgcagactttgtccagggtgatgcattcgccgctgtgacacttgaacttgttgggtccctcgcagagtgtcacattaacgcagccaacttcatcgctcatgtccttgcagtcatattcccggtcacactgccggctgccatggatgcagtttccatcagagcactggaattcgtcagggcgacaggtggccacagcgcagttttcctcgtcagatttgtccttgcagtcggggccaccatcacagcgccagctggagtggatgcactcgccacttaggcagtggaactcgaaggccgagcaggggctactgtccccttggaacacgtaaagacccctacagcgctgcggccactcatccgagccatcttcgcagtcggggtcgttgtcgcaggcccacagctgggggatgcaggtggagctgttgcactggaagctggcgggaccacaggtgagcaccgggcaggaggcctcgtctgagccgtccaagcagtcccggtctgagtcacagacgaactgccgagagatgcacttcccatcgtggcagcgaaactcgtcctgggagcacgtcttggggggacagccttgctcgtctgagccgttgtcgcagtccacttggccatcgcacctccagaactgaggaatgcagcggttgacacggcccccacagctgaagtccccggatttgcaggtgacagacaagcacgtctcctgggactcatcagagccatcctggcactcagcgctgccatcgcagacccacttgtaggagatgcatttcccgtcttggcactggaactcgtttctttcgcatctgtcgcccactgcagtccccgccgcggcgaggagcaaggcgacggtccagcgcaatttccagccccagggccccatgctcgcagcctctgccaggcagtgtcccgacccggatcacgacctgctgtgtcctagctggaaaccctggcttcccgcgattgcac

SEQ ID NO: 11309 - RNA, 3459 nt, Homo sapiens
  source 1..3459: mol_type = other RNA
ctgaatagctgggactacaggtgcccgccaccacgcccggctaattttttgtatttttagtagagacggggtttcacgtgttagccaggatggtctcgatctcctgacctcatgatccacccgcctcggcctcccaaagtgctgggattacaggcgtgagccactgcgcccggcctcaccgtgcatgttttaaacacatacccatcaacgacaagattggggaagtgaatggcttggaggcatttgcatagaagtggaagcactaggtgggcggacataaagacgacaatggcagttctcgatattcacgatcacggctttgaagtcccggtcaacctgcccctctctgtccccggcattcattgacacgggctttccctggcctgggatcccatcccaacacacacgacagaaaacagtgcaaaataataacacaaatgccaaatgtacacagtgtacaactctgaactgagaaagtgcaaggagaccacgggaatggaagtgggtaggggtcgggaggatgggcaccaggctggtgtcctgacagccacacctgggtgcaggccacgtgtcctcacggccaaggtaaccgggtgtctcaggcacttaataaatattaagggtgaccagtgactcaggctctgcctctgggaagtggcatcatttggtgaatgagtttggtctcggtgccaccacggattcagccagatcatttccgacgccatgaatccctttcctggcttaaggaaggtacaaacccacctcgaaagacactgggtgggtcatgattcgggggtgacagggcaaaggctaacctggctgtctagcaaggcttgcatagaagaggtaaacacgttgactcctgagtttaggggtttggcttagagattggtggatgaggcagggccagggggtcccgttggtgccatctgctgttgtgtgttgaaagccacttgcttctctgggcctgacatcccctcccctttcatcttccatgtttgaggattgtgtcacggtggagagaaactcaaaacttcctggagagaaatggaggtgtcatcctggtccccccgggcctgtttctcttatccttcacgaggaaaggaagaaaccaaaatcccaacccaagccattgcatgggcactgtccgaagcctgttctgcctcccagatgaataaatatataaaacaaagctctggcaggcaatgctttggtcttctctgtctttgaataaaacaaggccggcgaggtctcaggaagggttctgggcagggacgggactccaggcagatgttcacgccacgtcatcctccagactgaccatctgtctcgaggggtagctgtagccgtcctggttgtggcaaatgtggacctcatcctctgtggtcttctgatagacggggttgtcaaagttgatgctgttgatgttcttaagccgccagttcttccatagaaggaagacccccaggcaaaggaagacgaggagcacgatggggaggacaatggacagagccctcacgctactgggcttcttctcatttcctctgccagcaacgtcgcccagagcttggtgagacattgtcactatctccaccgtggtgagcccaggggtggccccaggcagccgggaggtgtcgggaacaggtcgggtggttgtgtgctgtgtccttacggctgtggagctgacctttagcctgacggtggatgtctcctgggtggccactgcagcctcagcctctgtgaggcagctcctcatgtccctggccagcagcatgccgtccgggcaggcgcaggtaaacttgggcgagtgggggttgatctgcggggcagggaggcacagatactggcagccgccattgctcagggtggtcctctcacaccagttcactcctcttggctgggtgaggttgtggaagagaaccatatcctctggggacagtaggttttcagccaacaagttgacatcggaacctgtgaggcggttggcactgaaaatggcttcgttgatgatatctgtccaaaatactttgtcctcaaagacggccaaggagaaggggtgggccagcctcttttcatcctccaagatggtcttccggttgcccccgttgacatcgatgcttgagatggagtgaagtttggagtcaacccagtagaggcggccactgaggagatctagggtgatgccattgggccactgaatgttttcagtcaccagcgagtagatgtccacaccattcaggccccctttcttgatcttggcgggagttccccagtcagtccagtacatgaagccatgaacaggatccaccacgatggcccttggcttggagccgttctccctgaataacgttttcctcttcacgcccttggtatccgcaacagagacagtgcccaggacagagtcggtccagtagatgttgctgtggatccagtccacagccagcccgtcgggggcctggatgtctctgctgatgacggtgtcataggaagagacgccgtgggctctgtcaagctgggtgctgcagatcattctctgggacaggtcagaccagtagattctattgctggccacctccgtgtccagagcgaccacgttcctcaggttggggatgaggctggtgtactcgctccggtccagcgtcatcttcctgacctcgtgccggttggtgaagaagaggtaggcgatggagcccacagccttgcaggccttcgtgtgggggtccagctggaagccttcctcacactggcacttgtagccaccctccaggttcacgcagagctggctgcaggtgtcgggatcctgacactcatcgatatcttcgcatcttcgctgggccaccagctggaagccgtcggggcacaggcactcgtagccgatcttaaggtcattgcagacgtgggaacagccgccgttgttgtccaagcattcgttggtcccgcactctttgatgggttcatctgaccagtcccggcagtctctagccatgttgcagactttgtccagggtgatgcattcgccgctgtgacacttgaacttgttgggtccctcgcagagtgtcagacagccttgctcgtctgagccgttgtcgcagtccacttggccatcgcacctccagaactgaggaatgcagcggttgacacggcccccacagctgaagtccccggatttgcaggtgacagacaagcacgtctcctgggactcatcagagccatcctggcactcagcgctgccatcgcagacccacttgtaggagatgcatttcccgtcttggcactggaactcgtttctttcgcatctgtcgcccactgcagtccccgccgcggcgaggagcaaggcgacggtccagcgcaatttccagccccagggccccatgctcgcagcctctgccaggcagtgtcccgacccggatcacgacctgctgtgtcctagctggaaaccctggcttcccgcgattgcac

SEQ ID NO: 11310 - RNA, 3916 nt, Homo sapiens
  source 1..3916: mol_type = other RNA
ctgaatagctgggactacaggtgcccgccaccacgcccggctaattttttgtatttttagtagagacggggtttcacgtgttagccaggatggtctcgatctcctgacctcatgatccacccgcctcggcctcccaaagtgctgggattacaggcgtgagccactgcgcccggcctcaccgtgcatgttttaaacacatacccatcaacgacaagattggggaagtgaatggcttggaggcatttgcatagaagtggaagcactaggtgggcggacataaagacgacaatggcagttctcgatattcacgatcacggctttgaagtcccggtcaacctgcccctctctgtccccggcattcattgacacgggctttccctggcctgggatcccatcccaacacacacgacagaaaacagtgcaaaataataacacaaatgccaaatgtacacagtgtacaactctgaactgagaaagtgcaaggagaccacgggaatggaagtgggtaggggtcgggaggatgggcaccaggctggtgtcctgacagccacacctgggtgcaggccacgtgtcctcacggccaaggtaaccgggtgtctcaggcacttaataaatattaagggtgaccagtgactcaggctctgcctctgggaagtggcatcatttggtgaatgagtttggtctcggtgccaccacggattcagccagatcatttccgacgccatgaatccctttcctggcttaaggaaggtacaaacccacctcgaaagacactgggtgggtcatgattcgggggtgacagggcaaaggctaacctggctgtctagcaaggcttgcatagaagaggtaaacacgttgactcctgagtttaggggtttggcttagagattggtggatgaggcagggccagggggtcccgttggtgccatctgctgttgtgtgttgaaagccacttgcttctctgggcctgacatcccctcccctttcatcttccatgtttgaggattgtgtcacggtggagagaaactcaaaacttcctggagagaaatggaggtgtcatcctggtccccccgggcctgtttctcttatccttcacgaggaaaggaagaaaccaaaatcccaacccaagccattgcatgggcactgtccgaagcctgttctgcctcccagatgaataaatatataaaacaaagctctggcaggcaatgctttggtcttctctgtctttgaataaaacaaggccggcgaggtctcaggaagggttctgggcagggacgggactccaggcagatgttcacgccacgtcatcctccagactgaccatctgtctcgaggggtagctgtagccgtcctggttgtggcaaatgtggacctcatcctctgtggtcttctgatagacggggttgtcaaagttgatgctgttgatgttcttaagccgccagttcttccatagaaggaagacccccaggcaaaggaagacgaggagcacttggtgagacattgtcactatctccaccgtggtgagcccaggggtggccccaggcagccgggaggtgtcgggaacaggtcgggtggttgtgtgctgtgtccttacggctgtggagctgacctttagcctgacggtggatgtctcctgggtggccactgcagcctcagcctctgtgaggcagctcctcatgtccctggccagcagcatgccgtccgggcaggcgcaggtaaacttgggcgagtgggggttgatctgcggggcagggaggcacagatactggcagccgccattgctcagggtggtcctctcacaccagttcactcctcttggctgggtgaggttgtggaagagaaccatatcctctggggacagtaggttttcagccaacaagttgacatcggaacctgtgaggcggttggcactgaaaatggcttcgttgatgatatctgtccaaaatactttgtcctcaaagacggccaaggagaaggggtgggccagcctcttttcatcctccaagatggtcttccggttgcccccgttgacatcgatgcttgagatggagtgaagtttggagtcaacccagtagaggcggccactgaggagatctagggtgatgccattgggccactgaatgttttcagtcaccagcgagtagatgtccacaccattcaggccccctttcttgatcttggcgggagttccccagtcagtccagtacatgaagccatgaacaggatccaccacgatggcccttggcttggagccgttctccctgaataacgttttcctcttcacgcccttggtatccgcaacagagacagtgcccaggacagagtcggtccagtagatgttgctgtggatccagtccacagccagcccgtcgggggcctggatgtctctgctgatgacggtgtcataggaagagacgccgtgggctctgtcaagctgggtgctgcagatcattctctgggacaggtcagaccagtagattctattgctggccacctccgtgtccagagcgaccacgttcctcaggttggggatgaggctggtgtactcgctccggtccagcgtcatcttcctgacctcgtgccggttggtgaagaagaggtaggcgatggagcccacagccttgcaggccttcgtgtgggggtccagctggaagccttcctcacactggcacttgtagccaccctccaggttcacgcagagctggctgcaggtgtcgggatcctgacactcatcgatatcttcgcatcttcgctgggccaccagctggaagccgtcggggcacaggcactcgtagccgatcttaaggtcattgcagacgtgggaacagccgccgttgttgtccaagcattcgttggtcccgcactctttgatgggttcatctgaccagtcccggcagtctctagccatgttgcagactttgtccagggtgatgcattcgccgctgtgacacttgaacttgttgggtccctcgcagagtgtcacattaacgcagccaacttcatcgctcatgtccttgcagtcatattcccggtcacactgccggctgccatggatgcagtttccatcagagcactggaattcgtcagggcgacaggtggccacagcgcagttttcctcgtcagatttgtccttgcagtcggggccaccatcacagcgccagctggagtggatgcactcgccacttaggcagtggaactcgaaggccgagcaggggctactgtccccttggaacacgtaaagacccctacagcgctgcggccactcatccgagccatcttcgcagtcggggtcgttgtcgcaggcccacagctgggggatgcaggtggagctgttgcactggaagctggcgggaccacaggtgagcaccgggcaggaggcctcgtctgagccgtccaagcagtcccggtctgagtcacagacgaactgccgagagatgcacttcccatcgtggcagcgaaactcgtcctgggagcacgtcttggggggacagccttgctcgtctgagccgttgtcgcagtccacttggccatcgcacctccagaactgaggaatgcagcggttgacacggcccccacagctgaagtccccggatttgcaggtgacagacaagcacgtctcctgggactcatcagagccatcctggcactcagcgctgccatcgcagacccacttgtaggagatgcatttcccgtcttggcactggaactcgtttctttcgcatctgtcgcccactgcagtccccgccgcggcgaggagcaaggcgacggtccagcgcaatttccagccccagggccccatgctcgcagcctctgccaggcagtgtcccgacccggatcacgacctgctgtgtcctagctggaaaccctggcttcccgcgattgcactcggggcccacgtcatttacagcatttcaat

SEQ ID NO: 11311 - RNA, 1164 nt, Homo sapiens
  source 1..1164: mol_type = other RNA
ctgaatagctgggactacaggtgcccgccaccacgcccggctaattttttgtatttttagtagagatggggtttcaccgtgttagccaggatggtctcgatctcctgatctcgtgatctgcccacctcagcctcccaaagtgctgggattacaggcatgagccaccgcgccgggccggaattattgttctttgctctcaattctgtatgacatctaagctccaaaaggaagaaggagaggctgggtaccctgtgccctgagctcagaacttcagggggatgaccggccagtacttgggctgctttcggtcacagtgcttgtcaaagctcagctgcaccgcggcctccatggcttggatcttggcagcactgtccccgtacaaacgcttcatctcggcctggcgccgctcaccaggcctctcagttggggcttctaccgaccggcgggtgttgcagtacaggtcgtggtcagcgttcacatagctgtccaggcgctctgcatccagctgctgctgccgccgtcgttcttctctatgcctctcggtctctgcaaagtactggcggagctcttcagtgatttccatattgctcaggtcacattctacctctgcatctgactcagtctccatctcttcctctttggacaaagcttggtcttcttttgtggatgcctggatcctactgctgtaacgtggatgctgcccagatcttctgaaatgtgaagaactgcaggggtagtcctgccaggccacatgatggtcatagaaggactgaggatacgcagcctcattatcgtaagagctttggggaagaagcgcagaaggtaagtaccatggaagattgaaacaggattccacggccttcctgtaggcattgtgatggctttgcatccaagccattgcttgatgataatgttgccagtatcttgcatataccggatgagaataccaaggcctggtagctttcgatgttgatgcctttaccgctgccatctctgattgtgaaagtccaaatgggtgctgaaactcgtgggcgcgcagcttgcggatcctgggcgttggccgcgcaggggcctagttttccttggagagacagagggggagtgggggacgcgagggaggcggctgttgccggggcgactggaagcgcgcttccggtgcggaac

SEQ ID NO: 11312 - RNA, 1136 nt, Homo sapiens
  source 1..1136: mol_type = other RNA
ctgaatagctgggactacaggtgcccgccaccacgcccggctaattttttgtatttttagtagagatggggtttcaccgtgttagccaggatggtctcgatctcctgatctcgtgatctgcccacctcagcctcccaaagtgctgggattacaggcatgagccaccgcgccgggccggaattattgttctttgctctcaattctgtatgacatctaagctcctgtgccctgagctcagaacttcagggggatgaccggccagtacttgggctgctttcggtcacagtgcttgtcaaagctcagctgcaccgcggcctccatggcttggatcttggcagcactgtccccgtacaaacgcttcatctcggcctggcgccgctcaccaggcctctcagttggggcttctaccgaccggcgggtgttgcagtacaggtcgtggtcagcgttcacatagctgtccaggcgctctgcatccagctgctgctgccgccgtcgttcttctctatgcctctcggtctctgcaaagtactggcggagctcttcagtgatttccatattgctcaggtcacattctacctctgcatctgactcagtctccatctcttcctctttggacaaagcttggtcttcttttgtggatgcctggatcctactgctgtaacgtggatgctgcccagatcttctgaaatgtgaagaactgcaggggtagtcctgccaggccacatgatggtcatagaaggactgaggatacgcagcctcattatcgtaagagctttggggaagaagcgcagaaggtaagtaccatggaagattgaaacaggattccacggccttcctgtaggcattgtgatggctttgcatccaagccattgcttgatgataatgttgccagtatcttgcatataccggatgagaataccaaggcctggtagctttcgatgttgatgcctttaccgctgccatctctgattgtgaaagtccaaatgggtgctgaaactcgtgggcgcgcagcttgcggatcctgggcgttggccgcgcaggggcctagttttccttggagagacagagggggagtgggggacgcgagggaggcggctgttgccggggcgactggaagcgcgcttccggtgcggaac

SEQ ID NO: 11313 - RNA, 2222 nt, Homo sapiens
  source 1..2222: mol_type = other RNA
ctgaatagctgggactacaggtgcccgccaccacgcccggctaattttttgtatttttagtagagatggggtttcaccgtgttagccaggatggtctcgatctcctgatctcgtgatctgcccacctcagcctcccaaagtgctgggattacaggcatgagccaccgcgccgggccggaattattgttctttgctctcaattctgtatgacatctaagctctgtagacataatgagataacaagaataaaaatgtcaggcaggtgattttcattccatgagaggtgcagttggcaaactaccatctgtagaccaaatctggcctgcagtctgtttttgtttttgttttgagacggagtcttgctctttctctaggttggagtgcagtggcgcgatctcagctcactgcaacctctgcctcctgggttcaagcaattcccctgcctcagtctcccacgtagctgggattacaggcacacaccaccatgcccggctcattttttgtattttagtagcgacgggtttcatcatgttggccaggatggtctccatctcctgacctcgtgatctgcccacctcggcctcccaaagtgctgggattacaggcatgaaccattgcgcccggccgcctgtttttataaataaagttttattagaacacagccacacccatttgtttacttactgtctacagctgctttcacactacaaagggagggttgagtagtcacaacactgaccgtgtggcttgcagtgccaaagatattcactctctggccctttatagaacatgcatccctctccactacaggtagtggtatttgtctcactacacacttggctcatttttagtgggggctaatggagctagagtcagagaggatatctggttttttaaaggcatttgtgtagttcagacaggttaaagacaagaaaagataaaaaagcaaaacaccaggcagtatctctaggcaagaacgttaatgaattgaactgttaccaacaacataaaaaaccagtatagtatatgcaaaattattttatgtcaggagaaaatttatcatgttggcaacagaacatgtcctgcagacctccaagtggctggcatagtacatccaccccgtgacaggcccactgggactgtggtgaacatgcctgtaccccagtacaaagtcccctttccctaagaaatgtacagaaggagagataaagagcgtgtacccaaaaggaagaaggagaggctgggtaccctgtgccctgagctcagaacttcagggggatgaccggccagtacttgggctgctttcggtcacagtgcttgtcaaagctcagctgcaccgcggcctccatggcttggatcttggcagcactgtccccgtacaaacgcttcatctcggcctggcgccgctcaccaggcctctcagttggggcttctaccgaccggcgggtgttgcagtacaggtcgtggtcagcgttcacatagctgtccaggcgctctgcatccagctgctgctgccgccgtcgttcttctctatgcctctcggtctctgcaaagtactggcggagctcttcagtgatttccatattgctcaggtcacattctacctctgcatctgactcagtctccatctcttcctctttggacaaagcttggtcttcttttgtggatgcctggatcctactgctgtaacgtggatgctgcccagatcttctgaaatgtgaagaactgcaggggtagtcctgccaggccacatgatggtcatagaaggactgaggatacgcagcctcattatcgtaagagctttggggaagaagcgcagaaggtaagtaccatggaagattgaaacaggattccacggccttcctgtaggcattgtgatggctttgcatccaagccattgcttgatgataatgttgccagtatcttgcatataccggatgagaataccaaggcctggtagctttcgatgttgatgcctttaccgctgccatctctgattgtgaaagtccaaatgggtgctgaaactccctgggaatgtctcccactcttttatggcacaagccttcagggactgaacagtaacttttctccaatgggctggtggagctcgtgggcgcgcagcttgcggatcctgggcgttggccgcgcaggggcctagttttccttggagagacagagggggagtgggggacgcgagggaggcggctgttgccggggcgact

SEQ ID NO: 11314 - RNA, 2140 nt, Homo sapiens
  source 1..2140: mol_type = other RNA
ctgaatagctgggactacaggtgcccgccaccacgcccggctaattttttgtatttttagtagagatggggtttcaccgtgttagccaggatggtctcgatctcctgatctcgtgatctgcccacctcagcctcccaaagtgctgggattacaggcatgagccaccgcgccgggccggaattattgttctttgctctcaattctgtatgacatctaagctctgtagacataatgagataacaagaataaaaatgtcaggcaggtgattttcattccatgagaggtgcagttggcaaactaccatctgtagaccaaatctggcctgcagtctgtttttgtttttgttttgagacggagtcttgctctttctctaggttggagtgcagtggcgcgatctcagctcactgcaacctctgcctcctgggttcaagcaattcccctgcctcagtctcccacgtagctgggattacaggcacacaccaccatgcccggctcattttttgtattttagtagcgacgggtttcatcatgttggccaggatggtctccatctcctgacctcgtgatctgcccacctcggcctcccaaagtgctgggattacaggcatgaaccattgcgcccggccgcctgtttttataaataaagttttattagaacacagccacacccatttgtttacttactgtctacagctgctttcacactacaaagggagggttgagtagtcacaacactgaccgtgtggcttgcagtgccaaagatattcactctctggccctttatagaacatgcatccctctccactacaggtagtggtatttgtctcactacacacttggctcatttttagtgggggctaatggagctagagtcagagaggatatctggttttttaaaggcatttgtgtagttcagacaggttaaagacaagaaaagataaaaaagcaaaacaccaggcagtatctctaggcaagaacgttaatgaattgaactgttaccaacaacataaaaaaccagtatagtatatgcaaaattattttatgtcaggagaaaatttatcatgttggcaacagaacatgtcctgcagacctccaagtggctggcatagtacatccaccccgtgacaggcccactgggactgtggtgaacatgcctgtaccccagtacaaagtcccctttccctaagaaatgtacagaaggagagataaagagcgtgtacccaaaaggaagaaggagaggctgggtaccctgtgccctgagctcagaacttcagggggatgaccggccagtacttgggctgctttcggtcacagtgcttgtcaaagctcagctgcaccgcggcctccatggcttggatcttggcagcactgtccccgtacaaacgcttcatctcggcctggcgccgctcaccaggcctctcagttggggcttctaccgaccggcgggtgttgcagtacaggtcgtggtcagcgttcacatagctgtccaggcgctctgcatccagctgctgctgccgccgtcgttcttctctatgcctctcggtctctgcaaagtactggcggagctcttcagtgatttccatattgctcaggtcacattctacctctgcatctgactcagtctccatctcttcctctttggacaaagcttggtcttcttttgtggatgcctggatcctactgctgtaacgtggatgctgcccagatcttctgaaatgtgaagaactgcaggggtagtcctgccaggccacatgatggtcatagaaggactgaggatacgcagcctcattatcgtaagagctttggggaagaagcgcagaaggtaagtaccatggaagattgaaacaggattccacggccttcctgtaggcattgtgatggctttgcatccaagccattgcttgatgataatgttgccagtatcttgcatataccggatgagaataccaaggcctggtagctttcgatgttgatgcctttaccgctgccatctctgattgtgaaagtccaaatgggtgctgaaactcgtgggcgcgcagcttgcggatcctgggcgttggccgcgcaggggcctagttttccttggagagacagagggggagtgggggacgcgagggaggcggctgttgccggggcgact

SEQ ID NO: 11315 - RNA, 2310 nt, Homo sapiens
  source 1..2310: mol_type = other RNA
ctgaatagctgggactacaggtgcccgccaccacgcccggctaattttttgtatttttagtagagatggggtttcaccgtgttagccaggatggtctcgatctcctgatctcgtgatctgcccacctcagcctcccaaagtgctgggattacaggcatgagccaccgcgccgggccggaattattgttctttgctctcaattctgtatgacatctaagctctgtagacataatgagataacaagaataaaaatgtcaggcaggtgattttcattccatgagaggtgcagttggcaaactaccatctgtagaccaaatctggcctgcagtctgtttttgtttttgttttgagacggagtcttgctctttctctaggttggagtgcagtggcgcgatctcagctcactgcaacctctgcctcctgggttcaagcaattcccctgcctcagtctcccacgtagctgggattacaggcacacaccaccatgcccggctcattttttgtattttagtagcgacgggtttcatcatgttggccaggatggtctccatctcctgacctcgtgatctgcccacctcggcctcccaaagtgctgggattacaggcatgaaccattgcgcccggccgcctgtttttataaataaagttttattagaacacagccacacccatttgtttacttactgtctacagctgctttcacactacaaagggagggttgagtagtcacaacactgaccgtgtggcttgcagtgccaaagatattcactctctggccctttatagaacatgcatccctctccactacaggtagtggtatttgtctcactacacacttggctcatttttagtgggggctaatggagctagagtcagagaggatatctggttttttaaaggcatttgtgtagttcagacaggttaaagacaagaaaagataaaaaagcaaaacaccaggcagtatctctaggcaagaacgttaatgaattgaactgttaccaacaacataaaaaaccagtatagtatatgcaaaattattttatgtcaggagaaaatttatcatgttggcaacagaacatgtcctgcagacctccaagtggctggcatagtacatccaccccgtgacaggcccactgggactgtggtgaacatgcctgtaccccagtacaaagtcccctttccctaagaaatgtacagaaggagagataaagagcgtgtacccaaaaggaagaaggagaggctgggtaccctgtgccctgagctcagaacttcagggggatgaccggccagtacttgggctgctttcggtcacagtgcttgtcaaagctcagctgcaccgcggcctccatggcttggatcttggcagcactgtccccgtacaaacgcttcatctcggcctggcgccgctcaccaggcctctcagttggggcttctaccgaccggcgggtgttgcagtacaggtcgtggtcagcgttcacatagctgtccaggcgctctgcatccagctgctgctgccgccgtcgttcttctctatgcctctcggtctctgcaaagtactggcggagctcttcagtgatttccatattgctcaggtcacattctacctctgcatctgactcagtctccatctcttcctctttggacaaagcttggtcttcttttgtggatgcctggatcctactgctgtaacgtggatgctgcccagatcttctgaaatgtgaagaactgcaggggtagtcctgccaggccacatgatggtcatagaaggactgaggatacgcagcctcattatcgtaagagctttggggaagaagcgcagaaggtaagtaccatggaagattgaaacaggattccacggccttcctgtaggcattgtgatggctttgcatccaagccattgcttgatgataatgttgccagtatcttgcatataccggatgagaataccaaggcctggtagctttcgatgttgatgcctttaccgctgccatctctgattgtgaaagtccaaatgggtgctgaaactctcaaagaaaagagagctgatggttgctgcagatttagatgccctttggtctttaatggtctttaattcgatctttcattcctcacctccctgggaatgtctcccactcttttatggcacaagccttcagggactgaacagtaacttttctccaatgggctggtggagctcgtgggcgcgcagcttgcggatcctgggcgttggccgcgcaggggcctagttttccttggagagacagagggggagtgggggacgcgagggaggcggctgttgccggggcgact

SEQ ID NO: 11316 - RNA, 1588 nt, Homo sapiens
  source 1..1588: mol_type = other RNA
ctgaatagctgggactacaggtgcccgccaccacgcccggctaattttttgtatttttttttagtacagacgggggtttcaccttgttagccaggatggtctcgatctcctgacctcgtgaatcgcccatcttggcctcctaaagtgctgggattacaggcattgagccaccgcacctggcccttctaccctcttatataccagttacctgttgtctcttcccccactagaaggtaagcttcatgagaacagaatttgtctttttccttgccgtttccctatttgagcaatgaattaaggaacctgtgagtagggatcaagctcctctttcacacagaagaaacacctggcctgggaggggtaaagggctttgtcgcagctggcgctgggtggagccggagtgtgaacagcgcccatcacagtgctcctcgcctcttccacccacccagaattctccccagtgacccaggaccaggcggctgccggggggccgagagccttcactaaatgtgacacatcagtgactacagccctgaaattcaaattggaagcctaggcttgtgctcatgtccagcaaatccaacaggtgaaaaatctagcttgtcagcttataatggttccattatcaaaagcttagccagggctgctggttttgtttttgtttagtttgaggctttttttttcttccaaatcatttctttttcccttatgagaacagtagaaaatatgggtaactatgcagtttatgtaagcattcaacaattgggagcgaattttctacaatcgcgagtgcggtcactgcgggaacgcatccgccccaggaaaggtgggcgggcagacgcgcgtgcgggcaaaaccgcaaggaggagcggctcggtggctccttctgcccgtgcgcccctgcttcccctcctcctgcttcaccgagatcaccaccggggctcctggaggtggcggtccccaggacactccgggagccggcggggtctcgctgggtcgctccgcccggaggctccccagacccctgcgcgcggcagccctggcccccgtcacccccgagcgcaagtcggcgaactccgagtggtcaggtcctccccaccgaggtgatttcggtccaacggcgatcggagtccccgaggacggtgcaggcgcctcccgcctccgtggggagcgcacagcagaaagcctactatgtgccaggtgccactgtgtcatttaatcctcttaccctgtcgcacacccggaggaggaaatcattgaccaggctctcgtgccggctgcagatgcttctctggaaggcactcttgagccagtcctcaatgctgcacacctgcacgcggctggagtgccagcagatggagaggctgcggagtgccgggcccaggaggaagttgtccttctggagttcagtgagggaacggaagtgcagcagggaccagagtgcggggtcctcaaacacgtcgtggagctgggagcaggtcctggcaaggctcttcctgctgtccttgtctaggaaggagaagaggtgcagcaggcactcccggttgagctgggttatgtgcatggtgagcagtggccacatgtgagt

SEQ ID NO: 11317 - RNA, 3599 nt, Homo sapiens
  source 1..3599: mol_type = other RNA
ctgaatagctgggactacaggtgcccgccaccacgcccggctaattttttgtatttttttttagtacagacgggggtttcaccttgttagccaggatggtctcgatctcctgacctcgtgaatcgcccatcttggcctcctaaagtgctgggattacaggcattgagccaccgcacctggcccttctaccctcttatataccagttacctgttgtctcttcccccactagaaggtaagcttcatgagaacagaatttgtctttttccttgccgtttccctatttgagcaatgaattaaggaacctgtgagtagggatcaagctcctctttcacacagaagaaacacctggcctgggaggggtaaagggctttgtcgcagctggcgctgggtggagccggagtgtgaacagcgcccatcacagtgctcctcgcctcttccacccacccagaattctccccagtgacccaggaccaggcggctgccggggggccgagagccttcactaaatgtgacacatcagtgactacagccctgaaattcaaattggaagcctaggcttgtgctcatgtccagcaaatccaacaggtgaaaaatctagcttgtcagcttataatggttccattatcaaaagcttagccagggctgctggttttgtttttgtttagtttgaggctttttttttcttccaaatcatttctttttcccttatgagaacagtagaaaatatgggtaactatgcagtttatgtaagcattcaacaattgggagcgaattttctacaatcgcgagtgcggtcactgcgggaacgcatccgccccaggaaaggtgggcgggcagacgcgcgtgcgggcaaaaccgcaaggaggagcggctcggtggctccttctgcccgtgcgcccctgcttcccctcctcctgcttcaccgagatcaccaccggggctcctggaggtggcggtccccaggacactccgggagccggcggggtctcgctgggtcgctccgcccggaggctccccagacccctgcgcgcggcagccctggcccccgtcacccccgagcgcaagtcggcgaactccgagtggtcaggtcctccccaccgaggtgatttcggtccaacggcgatcggagtccccgaggacggtgcaggcgcctcccgcctccgtggggagcgcacagcagaaagcctggggcggaagcaagaggggaaaggcggtggtgttgagtgagaaccagccgagtgttttccaaatatccatttaatcttgcgtttatcctatgtataaaatcgtaacgtgaggtaggctttcttatccccactgtgcagacggggaaaatgaggctcagaatatgcggtggtggtctgaaggtggaagagctgggttcgaagccaggacggtctggggctgcgctccttccccgggggcagcggcggggcggcgtctagcgctgcagcagcttgccgagggccgcggcgggcgcgcgcgggcgcgggggctggtcgggcagcatggcggcgctgtgctctgcccgcagggccaggcgcgggcacgcggcgcgcaggcggcgcaggccggccgcgctcacgttgcggcagaagtccacgtgcaatgtctgcagcgcgcgcccgtccgccgccacggcagccaacgtgcggttggtgacgcgcgcgcagttctccaggcgcagtgcgcgcaggcgtgggcagcagcgcagcaggcgcgccaggcagtcgtcggtaacgtggccgcagcccgagagcgtgacggacgccaggttggggcaccgaggaggactcgggccctgcgaggtgaagacacttggctgcgatgacactgcagggttccaagtcggctttctggccggcccattttccctcctctttctgcccctgcaccccaccgtaccttcatctgcgtgggttcttggctcgtagccttgggagcccctagtgggaagccccgaccccggcccagcagagtcctggggcggctgtggacagagggaatgccggttccaggagccacaacccttgactctttgtttcgctctggatgtgctgccttgcaggggagcggtgcttggcgattgctccagtctagcttcaagctgaggcccctgaatgtcccggcgggacgtgagtgggaagagggatttgtttccttggaggtggcctagtgacaggcccatcccaaccctcaaggcggtgggggcacgcgttagcattgagtccgggttcagcttagtagactagagctgttcctgcatcccctgggccaccagcctggaaaagggtagggttcggaggcagctagaggcaagccctgagcaggtacagtcacggacacccacccaggtcgcttggccagaaagcttgggggaccctctgctgcagcctcaccagcccctcccagcaaagaaaagatcttgagccaagttagacttggtttatcgccgtgtcagtcactcacggagccttcatttcctctgcgtggggggaataatgtctaccactggggttgtgaggagcctgcaacggggccttccacaggcagtcctaacccgctttccctggaaacaaacgggaccagcctgcttccagtccagaaggaccgactaatgggccggggccttggctccccgcagccagagggagctagagtctgggctggggaagcgtttccctttccctgccagcctcccccgcagctccgtgactgcccctggctgtgccagctcggctcctttgtgccaggggagggaagtaaggaacttaaatatgttgggtgcagccaggtgtcacaccgagcccgggcctccttcaggtttgtgtgccctcattagtcaccccgtcaacctctgcacccccagttttgtacatgaagaaactggctccggcagctcaggtgactggctggtgacttatttgctgtcagacccaggacagatgtctgaaccttgctgggcgtcacttcctcatttgtcaagtgggaggaattgttaccttcaaggtggttataaggattaggtgtttaagcctcaaaggtgttgggtgatcttttcttctaagaatctttggaataattctgatacagggaaaaaacaaagagcggactgtccccctgcccagccatcctcagccattcctcccgacctgagctgagtgccagaagaaccagattcagtagacgttcatcagtacctactatgtgccaggtgccactgtgtcatttaatcctcttaccctgtcgcacacccggaggaggaaatcattgaccaggctctcgtgccggctgcagatgcttctctggaaggcactcttgagccagtcctcaatgctgcacacctgcacgcggctggagtgccagcagatggagaggctgcggagtgccgggcccaggaggaagttgtccttctggagttcagtgagggaacggaagtgcagcagggaccagagtgcggggtcctcaaacacgtcgtggagctgggagcaggtcctggcaaggctcttcctgctgtccttgtctaggaaggagaagaggtgcagcaggcactcccggttgagctgggttatgtgcatggtgagcagtggccacatgt

SEQ ID NO: 11318 - RNA, 5011 nt, Homo sapiens
  source 1..5011: mol_type = other RNA
ctgaatagctgggactacaggtgcccgccaccacgcccggctaattttttgtatttttttttagtacagacgggggtttcaccttgttagccaggatggtctcgatctcctgacctcgtgaatcgcccatcttggcctcctaaagtgctgggattacaggcattgagccaccgcacctggcccttctaccctcttatataccagttacctgttgtctcttcccccactagaaggtaagcttcatgagaacagaatttgtctttttccttgccgtttccctatttgagcaatgaattaaggaacctgtgagtagggatcaagctcctctttcacacagaagaaacacctggcctgggaggggtaaagggctttgtcgcagctggcgctgggtggagccggagtgtgaacagcgcccatcacagtgctcctcgcctcttccacccacccagaattctccccagtgacccaggaccaggcggctgccggggggccgagagccttcactaaatgtgacacatcagtgactacagccctgaaattcaaattggaagcctaggcttgtgctcatgtccagcaaatccaacaggtgaaaaatctagcttgtcagcttataatggttccattatcaaaagcttagccagggctgctggttttgtttttgtttagtttgaggctttttttttcttccaaatcatttctttttcccttatgagaacagtagaaaatatgggtaactatgcagtttatgtaagcattcaacaattgggagcgaattttctacaatcgcgagtgcggtcactgcgggaacgcatccgccccaggaaaggtgggcgggcagacgcgcgtgcgggcaaaaccgcaaggaggagcggctcggtggctccttctgcccgtgcgcccctgcttcccctcctcctgcttcaccgagatcaccaccggggctcctggaggtggcggtccccaggacactccgggagccggcggggtctcgctgggtcgctccgcccggaggctccccagacccctgcgcgcggcagccctggcccccgtcacccccgagcgcaagtcggcgaactccgagtggtcaggtcctccccaccgaggtgatttcggtccaacggcgatcggagtccccgaggacggtgcaggcgcctcccgcctccgtggggagcgcacagcagaaagcctggggcggaagcaagaggggaaaggcggtggtgttgagtgagaaccagccgagtgttttccaaatatccatttaatcttgcgtttatcctatgtataaaatcgtaacgtgaggtaggctttcttatccccactgtgcagacggggaaaatgaggctcagaatatgcggtggtggtctgaaggtggaagagctgggttcgaagccaggacggtctggggctgcgctccttccccgggggcagcggcggggcggcgtctagcgctgcagcagcttgccgagggccgcggcgggcgcgcgcgggcgcgggggctggtcgggcagcatggcggcgctgtgctctgcccgcagggccaggcgcgggcacgcggcgcgcaggcggcgcaggccggccgcgctcacgttgcggcagaagtccacgtgcaatgtctgcagcgcgcgcccgtccgccgccacggcagccaacgtgcggttggtgacgcgcgcgcagttctccaggcgcagtgcgcgcaggcgtgggcagcagcgcagcaggcgcgccaggcagtcgtcggtaacgtggccgcagcccgagagcgtgacggacgccaggttggggcaccgaggaggactcgggccctgcgaggtgaagacacttggctgcgatgacactgcagggttccaagtcggctttctggccggcccattttccctcctctttctgcccctgcaccccaccgtaccttcatctgcgtgggttcttggctcgtagccttgggagcccctagtgggaagccccgaccccggcccagcagagtcctggggcggctgtggacagagggaatgccggttccaggagccacaacccttgactctttgtttcgctctggatgtgctgccttgcaggggagcggtgcttggcgattgctccagtctagcttcaagctgaggcccctgaatgtcccggcgggacgtgagtgggaagagggatttgtttccttggaggtggcctagtgacaggcccatcccaaccctcaaggcggtgggggcacgcgttagcattgagtccgggttcagcttagtagactagagctgttcctgcatcccctgggccaccagcctggaaaagggtagggttcggaggcagctagaggcaagccctgagcaggtacagtcacggacacccacccaggtcgcttggccagaaagcttgggggaccctctgctgcagcctcaccagcccctcccagcaaagaaaagatcttgagccaagttagacttggtttatcgccgtgtcagtcactcacggagccttcatttcctctgcgtggggggaataatgtctaccactggggttgtgaggagcctgcaacggggccttccacaggcagtcctaacccgctttccctggaaacaaacgggaccagcctgcttccagtccagaaggaccgactaatgggccggggccttggctccccgcagccagagggagctagagtctgggctggggaagcgtttccctttccctgccagcctcccccgcagctccgtgactgcccctggctgtgccagctcggctcctttgtgccaggggagggaagtaaggaacttaaatatgttgggtgcagccaggtgtcacaccgagcccgggcctccttcaggtttgtgtgccctcattagtcaccccgtcaacctctgcacccccagttttgtacatgaagaaactggctccggcagctcaggtgactggctggtgacttatttgctgtcagacccaggacagatgtctgaaccttgctgggcgtcacttcctcatttgtcaagtgggaggaattgttaccttcaaggtggttataaggattaggtgtttaagcctcaaaggtgttgggtgatcttttcttctaagaatctttggaataattctgatacagggaaaaaacaaagagcggactgtccccctgcccagccatcctcagccattcctcccgacctgagctgagtgccagaagaaccagattcagtagacgttcatcagtacctactatgtgccaggtgccactgtgtcatttaatcctcttaccctgttggataagaaaaatttagcacattttatagaagaagaaatgaggttgcaagagtttgaagtatttgagctggggtcacatggttggacgagctgagcggctcagcagagtgctgacagcaaagccctttgctctttatgtgacagcagggccccttgcttgatcagtacagtggcctgggaggtccacttcacaccttgcaggtttggggcattaagctcggttctcttacagtaagaatggaacaacttcaggacatgttgtgccattcgcctccccccaacccccacccatgtcactctagtctaattcctgggccttgttaagcccatcaaaatagccttgtccagtcggggcccaaccccaagtccatcttctgttttcttcctaccagctcaaaagaaaggtggggtcactacgctgtttccttccactcctgtcgtgctgccagcaaatagcagctatgaacttgggtggcagtaaactggctgagtctagttttccatgaacagccagggccagtttgttatatgatcaagggggtgtttttcctcaaaggcagcacgggactggcagaagctcagtgagaggctggttgaatagctctgtgttcttgcctgggccgctctgcccatgaggctgggaccatggagggagcctggcctggtggttcagtgtctatgtctgtgtctggggtgggggttagcagataaacacaagatgtatttgggacatacttacactaaaatattattcactgtttatctgaaattcatatttaactgggcagcctatatatttgctaaaatctggcaaccctagactgggcaaatcataccacctcgtggagcatcagtttgctaatttgaaaaattaggctaagccaccctccttaggaatactgtgtaaatcagtaattcatctactcctggagtctggtttggctcagctgacctgagcaccctggcttctccacctctggctccccaccctctctttcctccgtagtttcccaggccttgagggctgcttgctaggcctaatggaggggtgagctgattgctgcatctggaagccttttcccagagcctgaccttgaaaatccaggcccagctggacccacccagcacttaatgactaccagtacggaggccccacttcttggtgtttgcatgaagcagcccaggacctgtgaggctaagaggaggattagcaattgtttccctcatgattttattgtctcctggggaccctgctttgggcggtctggatgtctgccttgggcctagtttgaggcgccccgaaggtggagccatcttggtctcgtaatttgctcttccctgccccccaagagggaagccagagctagcggggccagcactgctcaggaggcaaggtggcctacctgtcgcacacccggaggaggaaatcattgaccaggctctcgtgccggctgcagatgcttctctggaaggcactcttgagccagtcctcaatgctgcacacctgcacgcggctggagtgccagcagatggagaggctgcggagtgccgggcccaggaggaagttgtccttctggagttcagtgagggaacggaagtgcagcagggaccagagtgcggggtcctcaaacacgtcgtggagctgggagcaggtcctggcaaggctcttcctgctgtccttgtctaggaaggagaagaggtgcagcaggcactcccggttgagctgggttatgtgcatggtgagcagtggccacatgtgagt

SEQ ID NO: 11319 - RNA, 2057 nt, Homo sapiens
  source 1..2057: mol_type = other RNA
ctgaatagctgggactacaggtgcccgccaccacgcccggctaattttttgtatttttttttagtacagacgggggtttcaccttgttagccaggatggtctcgatctcctgacctcgtgaatcgcccatcttggcctcctaaagtgctgggattacaggcattgagccaccgcacctggcccttctaccctcttatataccagttacctgttgtctcttcccccactagaaggtaagcttcatgagaacagaatttgtctttttccttgccgtttccctatttgagcaatgaattaaggaacctgtgagtagggatcaagctcctctttcacacagaagaaacacctggcctgggaggggtaaagggctttgtcgcagctggcgctgggtggagccggagtgtgaacagcgcccatcacagtgctcctcgcctcttccacccacccagaattctccccagtgacccaggaccaggcggctgccggggggccgagagccttcactaaatgtgacacatcagtgactacagccctgaaattcaaattggaagcctaggcttgtgctcatgtccagcaaatccaacaggtgaaaaatctagcttgtcagcttataatggttccattatcaaaagcttagccagggctgctggttttgtttttgtttagtttgaggctttttttttcttccaaatcatttctttttcccttatgagaacagtagaaaatatgggtaactatgcagtttatgtaagcattcaacaattgggagcgaattttctacaatcgcgagtgcggtcactgcgggaacgcatccgccccaggaaaggtgggcgggcagacgcgcgtgcgggcaaaaccgcaaggaggagcggctcggtggctccttctgcccgtgcgcccctgcttcccctcctcctgcttcaccgagatcaccaccggggctcctggaggtggcggtccccaggacactccgggagccggcggggtctcgctgggtcgctccgcccggaggctccccagacccctgcgcgcggcagccctggcccccgtcacccccgagcgcaagtcggcgaactccgagtggtcaggtcctccccaccgaggtgatttcggtccaacggcgatcggagtccccgaggacggtgcaggcgcctcccgcctccgtggggagcgcacagcagaaagcctggggcggaagcaagaggggaaaggcggtggtgttgagtgagaaccagccgagtgttttccaaatatccatttaatcttgcgtttatcctatgtataaaatcgtaacgtgaggtaggctttcttatccccactgtgcagacggggaaaatgaggctcagaatatgcggtggtggtctgaaggtggaagagctgggttcgaagccaggacggtctggggctgcgctccttccccgggggcagcggcggggcggcgtctagcgctgcagcagcttgccgagggccgcggcgggcgcgcgcgggcgcgggggctggtcgggcagcatggcggcgctgtgctctgcccgcagggccaggcgcgggcacgcggcgcgcaggcggcgcaggccggccgcgctcacgttgcggcagaagtccacgtgcaatgtctgcagcgcgcgcccgtccgccgccacggcagccaacgtgcggttggtgacgcgcgcgcagttctccaggcgcagtgcgcgcaggcgtgggcagcagcgcagcaggcgcgccaggcagtcgtcggtaacgtggccgcagcccgagagcgtgacggacgccaggttggggcacctactatgtgccaggtgccactgtgtcatttaatcctcttaccctgtcgcacacccggaggaggaaatcattgaccaggctctcgtgccggctgcagatgcttctctggaaggcactcttgagccagtcctcaatgctgcacacctgcacgcggctggagtgccagcagatggagaggctgcggagtgccgggcccaggaggaagttgtccttctggagttcagtgagggaacggaagtgcagcagggaccagagtgcggggtcctcaaaca

SEQ ID NO: 11320 - RNA, 3595 nt, Homo sapiens
  source 1..3595: mol_type = other RNA
ctgaatagctgggactacaggtgcccgccaccacgcccggctaattttttgtatttttttttagtacagacgggggtttcaccttgttagccaggatggtctcgatctcctgacctcgtgaatcgcccatcttggcctcctaaagtgctgggattacaggcattgagccaccgcacctggcccttctaccctcttatataccagttacctgttgtctcttcccccactagaaggtaagcttcatgagaacagaatttgtctttttccttgccgtttccctatttgagcaatgaattaaggaacctgtgagtagggatcaagctcctctttcacacagaagaaacacctggcctgggaggggtaaagggctttgtcgcagctggcgctgggtggagccggagtgtgaacagcgcccatcacagtgctcctcgcctcttccacccacccagaattctccccagtgacccaggaccaggcggctgccggggggccgagagccttcactaaatgtgacacatcagtgactacagccctgaaattcaaattggaagcctaggcttgtgctcatgtccagcaaatccaacaggtgaaaaatctagcttgtcagcttataatggttccattatcaaaagcttagccagggctgctggttttgtttttgtttagtttgaggctttttttttcttccaaatcatttctttttcccttatgagaacagtagaaaatatgggtaactatgcagtttatgtaagcattcaacaattgggagcgaattttctacaatcgcgagtgcggtcactgcgggaacgcatccgccccaggaaaggtgggcgggcagacgcgcgtgcgggcaaaaccgcaaggaggagcggctcggtggctccttctgcccgtgcgcccctgcttcccctcctcctgcttcaccgagatcaccaccggggctcctggaggtggcggtccccaggacactccgggagccggcggggtctcgctgggtcgctccgcccggaggctccccagacccctgcgcgcggcagccctggcccccgtcacccccgagcgcaagtcggcgaactccgagtggtcaggtcctccccaccgaggtgatttcggtccaacggcgatcggagtccccgaggacggtgcaggcgcctcccgcctccgtggggagcgcacagcagaaagcctggggcggaagcaagaggggaaaggcggtggtgttgagtgagaaccagccgagtgttttccaaatatccatttaatcttgcgtttatcctatgtataaaatcgtaacgtgaggtaggctttcttatccccactgtgcagacggggaaaatgaggctcagaatatgcggtggtggtctgaaggtggaagagctgggttcgaagccaggacggtctggggctgcgctccttccccgggggcagcggcggggcggcgtctagcgctgcagcagcttgccgagggccgcggcgggcgcgcgcgggcgcgggggctggtcgggcagcatggcggcgctgtgctctgcccgcagggccaggcgcgggcacgcggcgcgcaggcggcgcaggccggccgcgctcacgttgcggcagaagtccacgtgcaatgtctgcagcgcgcgcccgtccgccgccacggcagccaacgtgcggttggtgacgcgcgcgcagttctccaggcgcagtgcgcgcaggcgtgggcagcagcgcagcaggcgcgccaggcagtcgtcggtaacgtggccgcagcccgagagcgtgacggacgccaggttggggcacctactatgtgccaggtgccactgtgtcatttaatcctcttaccctgttggataagaaaaatttagcacattttatagaagaagaaatgaggttgcaagagtttgaagtatttgagctggggtcacatggttggacgagctgagcggctcagcagagtgctgacagcaaagccctttgctctttatgtgacagcagggccccttgcttgatcagtacagtggcctgggaggtccacttcacaccttgcaggtttggggcattaagctcggttctcttacagtaagaatggaacaacttcaggacatgttgtgccattcgcctccccccaacccccacccatgtcactctagtctaattcctgggccttgttaagcccatcaaaatagccttgtccagtcggggcccaaccccaagtccatcttctgttttcttcctaccagctcaaaagaaaggtggggtcactacgctgtttccttccactcctgtcgtgctgccagcaaatagcagctatgaacttgggtggcagtaaactggctgagtctagttttccatgaacagccagggccagtttgttatatgatcaagggggtgtttttcctcaaaggcagcacgggactggcagaagctcagtgagaggctggttgaatagctctgtgttcttgcctgggccgctctgcccatgaggctgggaccatggagggagcctggcctggtggttcagtgtctatgtctgtgtctggggtgggggttagcagataaacacaagatgtatttgggacatacttacactaaaatattattcactgtttatctgaaattcatatttaactgggcagcctatatatttgctaaaatctggcaaccctagactgggcaaatcataccacctcgtggagcatcagtttgctaatttgaaaaattaggctaagccaccctccttaggaatactgtgtaaatcagtaattcatctactcctggagtctggtttggctcagctgacctgagcaccctggcttctccacctctggctccccaccctctctttcctccgtagtttcccaggccttgagggctgcttgctaggcctaatggaggggtgagctgattgctgcatctggaagccttttcccagagcctgaccttgaaaatccaggcccagctggacccacccagcacttaatgactaccagtacggaggccccacttcttggtgtttgcatgaagcagcccaggacctgtgaggctaagaggaggattagcaattgtttccctcatgattttattgtctcctggggaccctgctttgggcggtctggatgtctgccttgggcctagtttgaggcgccccgaaggtggagccatcttggtctcgtaatttgctcttccctgccccccaagagggaagccagagctagcggggccagcactgctcaggaggcaaggtggcctacctgtcgcacacccggaggaggaaatcattgaccaggctctcgtgccggctgcagatgcttctctggaaggcactcttgagccagtcctcaatgctgcacacctgcacgcggctggagtgccagcagatggagaggctgcggagtgccgggcccaggaggaagttgtccttctggagttcagtgagggaacggaagtgcagcagggaccagagtgcggggtcctcaaacacgtcgtggagctgggagcaggtcctggcaaggctcttcctgctgtccttgtctaggaaggagaagaggtgcagcaggcactcccggttgagctgggttatgtgcatggtgagcagtggccacatgtgagt

SEQ ID NO: 11321 - RNA, 1545 nt, Homo sapiens
  source 1..1545: mol_type = other RNA
ctgaatagctgggactacaggtgcccgccaccacgcccggctaattttttgtatttttttttagtacagacgggggtttcaccttgttagccaggatggtctcgatctcctgacctcgtgaatcgcccatcttggcctcctaaagtgctgggattacaggcattgagccaccgcacctggcccttctaccctcttatataccagttacctgttgtctcttcccccactagaaggtaagcttcatgagaacagaatttgtctttttccttgccgtttccctatttgagcaatgaattaaggaacctgtgagtagggatcaagctcctctttcacacagaagaaacacctggcctgggaggggtaaagggctttgtcgcagctggcgctgggtggagccggagtgtgaacagcgcccatcacagtgctcctcgcctcttccacccacccagaattctccccagtgacccaggaccaggcggctgccggggggccgagagccttcactaaatgtgacacatcagtgactacagccctgaaattcaaattggaagcctaggcttgtgctcatgtccagcaaatccaacaggtgaaaaatctagcttgtcagcttataatggttccattatcaaaagcttagccagggctgctggttttgtttttgtttagtttgaggctttttttttcttccaaatcatttctttttcccttatgagaacagtagaaaatatgggtaactatgcagtttatgtaagcattcaacaattgggagcgaattttctacaatcgcgagtgcggtcactgcgggaacgcatccgccccaggaaaggtgggcgggcagacgcgcgtgcgggcaaaaccgcaaggaggagcggctcggtggctccttctgcccgtgcgcccctgcttcccctcctcctgcttcaccgagatcaccaccggggctcctggaggtggcggtccccaggacactccgggagccggcggggtctcgctgggtcgctccgcccggaggctccccagacccctgcgcgcggcagccctggcccccgtcacccccgagcgcaagtcggcgaactccgagtggtcaggtcctccccaccgaggtgatttcggtccaacggcgatcggagtccccgaggacggtgcaggcgcctcccgcctccgtggggagcgcacagcagaaagcctgtcgcacacccggaggaggaaatcattgaccaggctctcgtgccggctgcagatgcttctctggaaggcactcttgagccagtcctcaatgctgcacacctgcacgcggctggagtgccagcagatggagaggctgcggagtgccgggcccaggaggaagttgtccttctggagttcagtgagggaacggaagtgcagcagggaccagagtgcggggtcctcaaacacgtcgtggagctgggagcaggtcctggcaaggctcttcctgctgtccttgtctaggaaggagaagaggtgcagcaggcactcccggttgagctgggttatgtgcatggtgagcagtggccacatgtgagt

SEQ ID NO: 11322 - RNA, 1699 nt, Homo sapiens
  source 1..1699: mol_type = other RNA
ctgaatagctgggactacaggtgcccgccaccacgcccggctaattttttgtattttttttttttttagtagagacggggtttcaccatagccaggatggtcttgatctcctgacctcgtgatccgcctgcctcggcctcccaaagtgctgggattacaggcgtgagccactgcgcccggccctcctgctgtgaattttctgaaccatgtatgtgaattaatttgcacaggttttcccccattacttagatgtacaggatttctttcctgtgtgacttctcacatgaccttgaaaggctttgggacaactgaaagctttcccacatttttcgcatttactgggcttctgtccaatctgcgttcttacatttttggaagagcaaagcccgcctgaaggttttcccacactggctgcatttacaggtttctccccagtgtgctttctctcatgtttgtgtaaagatgaggaccaaccatacgttttcccacacgtttcacatttatagactttctctctagtttgtgatttgacatctgtggaggggcgaggcctcgcggaagactttcccacgctgcccccactcacaggtttctttttagcatgcgttctcgcgtgtttgtgtaaggatgagggccaaccgaatgctttcccgcattttccacacttatagggtttctccccgttgtgaattctcacgtgtcgttgaaaggatgttgcccagcagtaggctttcccacactgcttgcactcatacggtctccctccggcgtgcatgatcatatggactcgaaaggatttctgacacctgaaggctttcccacagtgcttgcactcatacggtctccctccggcgtgcatcatcacatgtgcgcgaaaggatttgggacaactgaagcctttcccacactgcccacattcgtagggtttctctccagtgtgagtccttacatgttcagtgagagagtgggaacgaagaaatgtcttcccgcaagattgacaggcatagggtttctctccactgtgagttttctcatgcgtctgtaggtaggaagggcgactgaaggctttcccacattccttacatttatataatttttgtccagagtgagctcttttgtgccttatcagggatgaggaatgggtgaagagttttccacactgactgcattcgtaccgtcttacactagtacaacaattcttgcgcagatgacgattacaatttcgagtctttctgaaggttcttccacgtttattacctttactgcttttacatggtctctccacccttggatttctgctcaaatgtctctccttggtgttgtgcttgtctttaacgctatgttcttcccaattttttcctaaaagggaggcccatatattctttcttgtgaacttttctattttctgtttgagggataatttttctccagaagtatcctgctgagaaatagacccactggctttaagctgagcctcattatctactgaggccaggtgcttgaaggtctccagcatgacatctctgtagagttttctctgagcaggattcagcaaggcccactcctccagcgtgaaatccacaaccacgtcttcaaagaccactgtgtccatgtcctgtccgttcctgagctctttgaggagctccctgctcctcgcagccggtgcaggtgagcacgacggggacacctgtggtcactc

SEQ ID NO: 11323 - RNA, 1695 nt, Homo sapiens
  source 1..1695: mol_type = other RNA
ctgaatagctgggactacaggtgcccgccaccacgcccggctaattttttgtattttttttttttttagtagagacggggtttcaccatagccaggatggtcttgatctcctgacctcgtgatccgcctgcctcggcctcccaaagtgctgggattacaggcgtgagccactgcgcccggccctcctgctgtgaattttctgaaccatgtatgtgaattaatttgcacaggttttcccccattacttagatgtacaggatttctttcctgtgtgacttctcacatgaccttgaaaggctttgggacaactgaaagctttcccacatttttcgcatttactgggcttctgtccaatctgcgttcttacatttttggaagagcaaagcccgcctgaaggttttcccacactggctgcatttacaggtttctccccagtgtgctttctctcatgtttgtgtaaagatgaggaccaaccatacgttttcccacacgtttcacatttatagactttctctctagtttgtgatttgacatctgtggaggggcgaggcctcgcggaagactttcccacgctgcccccactcacaggtttctttttagcatgcgttctcgcgtgtttgtgtaaggatgagggccaaccgaatgctttcccgcattttccacacttatagggtttctccccgttgtgaattctcacgtgtcgttgaaaggatgttgcccagcagtaggctttcccacactgcttgcactcatacggtctccctccggcgtgcatgatcatatggactcgaaaggatttctgacacctgaaggctttcccacagtgcttgcactcatacggtctccctccggcgtgcatcatcacatgtgcgcgaaaggatttgggacaactgaagcctttcccacactgcccacattcgtagggtttctctccagtgtgagtccttacatgttcagtgagagagtgggaacgaagaaatgtcttcccgcaagattgacaggcatagggtttctctccactgtgagttttctcatgcgtctgtaggtaggaagggcgactgaaggctttcccacattccttacatttatataatttttgtccagagtgagctcttttgtgccttatcagggatgaggaatgggtgaagagttttccacactgactgcattcgtaccgtcttacactagtacaacaattcttgcgcagatgacgattacaatttcgagtctttctgaaggttcttccacgtttattacctttactgcttttacatggtctctccacccttggatttctgctcaaatgtctctccttggtgttgtgcttgtctttaacgctatgttcttcccaattttttcctaaaagggaggcccatatattctttcttgtgaacttttctattttctgtttgagggataatttttctccagaagtatcctgctgagaaatagacccactggctttaagctgagcctcattattgaggccaggtgcttgaaggtctccagcatgacatctctgtagagttttctctgagcaggattcagcaaggcccactcctccagcgtgaaatccacaaccacgtcttcaaagaccactgtgtccatgtcctgtccgttcctgagctctttgaggagctccctgctcctcgcagccggtgcaggtgagcacgacggggacacctgtggtcactc

SEQ ID NO: 11324 - RNA, 62 nt, Homo sapiens
  source 1..62: mol_type = other RNA
ctgaatagctgggactacaggtgcccgccaccacgcccggctaatttttttgtatttttagt

SEQ ID NO: 11325 - RNA, 6392 nt, Homo sapiens
  source 1..6392: mol_type = other RNA
ctgaatagctgggactacaggtgcccgccaccacgcccggctaattttttttgtatttttagtagagacggggtttcaccatgttgggctcgatctcctgacctcatgatccgcccgcctcggcctcccaaagtgctgggattacaggcgtgatgagccacctagtgctaattcatctctaaacctctgtagttggagtctcctgaaatctcagactacctcctgctttcattttctacccagggaatacactattgtcctaagttatttagccttgaaatgtcagaggcattttaggttcttcatgtttctcccactttcagttgattaccattacaggatcttaggcttctttttatctttttgcagtgccttgcatccactggttgtttgttttttctgttgggcactacttatttccttacctctggtttcttctcctacagcttatgttctgaaatgtgtattcctaaaatactgttttcctcttgttacttttctgctcgaggacttccagtaacttaccattgtttataaggtgatgttcaaacccttcagtctggagactttctgccacctatctgactgtacctttatcttcaagcttatctctttccaaacaagaggctcatttagcagctttctctgattgccatgttcatcctacactcagcctcattcagtttacagcatggaaactgtataggacctctttcctatagaaattgaagacacttaaataggaagaaaattaaaatatacatttggatacatgagtattccagtcaaataatatctataaaataccagatagagtataaaagacaactgaaggacaacagagtgatgaaaggactttattaggcatttggatttggttatgatttaaatttcaatttaattagaacgtttccatggcaaggaaggaagcatggaggactgtggaaaagtcattcagtattgagttcatttgcattagaggaatttcatagtttaaaacttgtatatctttacctatccttcgtatgttttcttcttaagcatatttgactttttctacctcagcatctgtataagaaaatatttgtgagtcagatgtttgtgggttttccttacctattattattttcttccatgctttacaacacattttttaaactaccttgttcttaaataattacacggacctgcttctgtgtactttcacagaatctttgacagttaaaaattgtatgttatataaaaatttgacaagcttctacagttaggaaaagcctttagaaatctgccttccccaaaccgtatgttatcatagcactcatgtctccccatgtctaaaaggtaaatagatacagaaacctcaccaaaagttgaatcatctgtactaaaccactgcttttttatccagactttttatataaatcttttattttccaaaaaactgatcttttacctacccctcttagagttaaaaatattgcctgtcaggcaagagtatagtatgccaatataaataatatgctttatttggttagaaacagttggtttgggaagctagcaacatagcatattctttacaaatttaataaggtgtattttgatactgtgataacctgcattgtaaattaccaaatggttggaattgaccagtttatacttattaaaatttttgatgtgccaatggctatccaattcattgcatttgtgaattgtgcttttagaaaaattgtggacattttagttttatatacatatttatgagttatttgtgcatatgataaaattatatataataataaaagtatatatgtaacttacattgtgcccttgattattgaaaacttcctttttataacagattcactgtttggaagctaaagtaaaaatgagccatgttaccagaagtaataatttctatcttattactgatgtttttatactttgtggtaaaactatggaaagttaggttttcagatgctgtggtagctgaaagagtttgatgtacatgtggttaaagtgtgaagaaaatatgaaggaaaaagtatgaaaagtaccctagtcattacctaattgctattttgtttttaaggatctaagaagtgttattgcattgtacagattattttagaaattcacatctttgctggcttttcctttaacaccaagaatatctgttatcatctgtttggtactgtgttttgtttcctcttttaaagtaaaatattgaagtgatatttaaatgtttgcaagtctcatgaccttcctatagaaattcacattagtataataatttacattacaaatacaatatagcctttaattttgaagagtaaaaatggaaatggaagatgaattactatagtgtagttcacttaaatcgaaaatgtatatttgaatagtttcagtgaaatttggctcatatgaccatagtttaatagaattcttatttctattattgataaccttgaataaaaggatctaattataagttatctaggttttttcccttttagggaagagatgttatgtttttgtactactcttggctatagctgtaaaggatgtgtctgaacctggtaaaactttttaaaattctgagttcagttctgtaatattaatgaatattacattataaagatcacttaggaggggtttaatatatgctgatttgttttatatgaattgttagaaatatatacagaaataagggtagtttcaggctacctttcaggctattattagttgggcaagcttatttttagagcttttccctttcattggttggatgtagggcctgggaatacaaatagattttaatagttttactaggtaaaactgctagagagaaaattcatgtcccaagtagaaaaattaatatagctgaatacttaagtccttgttgaaaagttttctgaaatactggagttcattttcctgccttggtaaggcatttttaaaatttagtttagatggcttaaaccatttaaagaagctgtcttcattgtaaatatcaattgtcaatatcaattttcactgttcagaactgtccaaatactcttaaggtttgtctatactaaattcctattctttttaaaatttacctgttttccttctccctagtcccctttcctgccctttaaatctgaataaccagaagccatatattcaatgttttatgtattttcaatgttttgtgtataacgatatatgaagttagtgaattctgtaagacaaaaagatcgtttttattcacttttgattacaaaaaaaggttacatgaataaaataacaatttcctttaagagagggattcctgaatgattaaactgccaaggaaaaaagagtgaattcttccttttaataaaggtgacctaggtcctgaggaagttaggaaaaaagaaaaactcacattatacttgttaaatttgttttcaaatgtgattattaagttgttgtatttattttttgttatagacaaagcaaacccaaaaactagtctaaaaaagaattcctatgcattattaaaagagatagtaataaaatatgtattggtggtgaagaattccacaagcactcaagattgacataacctttaacaaagtggaaaaacttttattagaactgccaattctaggttcaaatttatgtcaaagcactttatggtaccataattagtacaactaaattattttttagctttaaatgtcatttttcactaaatgattttaaataagacatctgagagttacttgaggcaagtttagatacctgtacaagtttagattttgagaaactccctatttcctcattgtgtgtctctttcacatgctttttagaatcatttattccacaacatgtttccaaattctatctagtaatttttaaacttcaaaaataatctccctgttcaattacaaggttctaaagacaataaaataccttataatttcagtaacaacatttttctttttcttgggcaaagtattacaaagtgttcgcctaatcctcataatgttcttttaaattaacgtggaaatcagtaattatcctccttaaaaggtgggaaaactgaagcactgtaaagttaggttctgacccaaggtcagagtaaccaaggtgaaaaatctgggtatttcaacaactgctgttccagtgtatgtctattattattcgtatcaccttgaataaaatatggcatttaaaaatttatgatgtcataatgctgagtgagtctctactgagcagggctgcataatgttaaattttaaaaagaaaaattacaagcccggctttaaataataaagggattaagtacagaatatatatatttttaagatcatcgatgccattgtgtccaataaattgccttactaacagtgttatgttgtcttaagacagtgctgattagaaaaagtgtacaaagaatgctctaaagacccatggaacacaatataccttaaattggcactaagctataccacaataaaagtcatacatattgaatgttgacatacactgagaagggtgacgagttttcaataacgtattttagaaaattgttcattttttgcttaaatttatccgaatataagacctataaagcaagacaaggaagcatggagcactgagtcttttcatgcccagtatccaacagtcagagctatgttttcctcctgttcatgatggcttggcttttcagatggtgccaatcctgtgatgaggcacttgaagagtttgaaggttagggcatgtaaaatatggagctggaaggaagcatgctgctattccattggaagcaaaagggagtgtaggcccatagaatacttcttctttgccttctctgcttacatccagtacctggatacaagccagaggctcatttgtccaaattgaatatccaccaactaaatatattctcccattatggacagcaactccagattcattttggccagtcagcaggttgaaattacaacgtgtccactggtcagtgtctatgttgtaagaatctatatggcgcacaaggatccggtcattattgtagtctaggtcattgcctccaagaacataaagcttcctttgtacagcagccatggaatggtagacccttctctgcagcatggggctacggcttatccacttattctggttaggttcatacaccattagcctgttctgatattgtgccgtattagttactccacctgatatccaaagaagaccatcagccacatatccagcatggcatgaaagggatctgtcaaaggactgaacaaaagtccatttgttcttcttggggcaatatcgctcaactgtaggcagaacctggcgcagttcatttctgcccccaactgcatagaggtattcctccatggcacccagcacaaaatgctcccggcagtttttcatgggtgctatctctgcccaggaattactgcgggggtcatagcgacaggcagtcctcacagcacacgtccggccactggcatgctcaacttcccctcctgccacaaacaggaagtcccccatgactgccacacaatggtggctccttcccacaggcatgggagccagctcactccagttggcaatggcagctatgagagcattctcctgatcaacaggattgaagtaccgaagttccttgaccttgcagacctcgcgctttttcccaccaatgatatacagagtgtctgactggaatcgtggtttggtcctgcgagtctgccagacaggctgtgcatagatgctctggtggtattccagggcctcgttgacaagggctgttgcagtctcacttgcttggacaagggggtgggacagggcaactgtatggagagtatccacatccattaggccaaagcggatgtattgcaggagctcgtccatgtactggtagtggcagttgtgttccaaccacctcacagctagcagtcttgtcatcccattgaggtaagccagggcaccagtctcccctcagtgcacaaaaggcagcacaaattccacacttctgccagatctgctcttcactcagggaggtcaggcggtcgctcttcagcacctcctgaagcaggcaatagggaagcgttagaacttcttctgggcggctcttcaggagttcagagagatgtttcactaagaaatcgatcactgccttctccaacaaagtgaggttaaagaggtcagcaagtctgtacagatccaagtaattaaagctatttaattcctggatgagatagtgggagcataaattgagaagctccaacagctgtaggtgactgcccgctgctagcacatcctggatcacacctggctccagcaaaatctgtcctgtgtatgcaaactccagagcctgctttaagccaaggctggtcacaccgtgcaaattaacc

SEQ ID NO: 11326 - RNA, 6435 nt, Homo sapiens
  source 1..6435: mol_type = other RNA
ctgaatagctgggactacaggtgcccgccaccacgcccggctaattttttttgtatttttagtagagacggggtttcaccatgttgggctcgatctcctgacctcatgatccgcccgcctcggcctcccaaagtgctgggattacaggcgtgatgagccacctagtgctaattcatctctaaacctctgtagttggagtctcctgaaatctcagactacctcctgctttcattttctacccagggaatacactattgtcctaagttatttagccttgaaatgtcagaggcattttaggttcttcatgtttctcccactttcagttgattaccattacaggatcttaggcttctttttatctttttgcagtgccttgcatccactggttgtttgttttttctgttgggcactacttatttccttacctctggtttcttctcctacagcttatgttctgaaatgtgtattcctaaaatactgttttcctcttgttacttttctgctcgaggacttccagtaacttaccattgtttataaggtgatgttcaaacccttcagtctggagactttctgccacctatctgactgtacctttatcttcaagcttatctctttccaaacaagaggctcatttagcagctttctctgattgccatgttcatcctacactcagcctcattcagtttacagcatggaaactgtataggacctctttcctatagaaattgaagacacttaaataggaagaaaattaaaatatacatttggatacatgagtattccagtcaaataatatctataaaataccagatagagtataaaagacaactgaaggacaacagagtgatgaaaggactttattaggcatttggatttggttatgatttaaatttcaatttaattagaacgtttccatggcaaggaaggaagcatggaggactgtggaaaagtcattcagtattgagttcatttgcattagaggaatttcatagtttaaaacttgtatatctttacctatccttcgtatgttttcttcttaagcatatttgactttttctacctcagcatctgtataagaaaatatttgtgagtcagatgtttgtgggttttccttacctattattattttcttccatgctttacaacacattttttaaactaccttgttcttaaataattacacggacctgcttctgtgtactttcacagaatctttgacagttaaaaattgtatgttatataaaaatttgacaagcttctacagttaggaaaagcctttagaaatctgccttccccaaaccgtatgttatcatagcactcatgtctccccatgtctaaaaggtaaatagatacagaaacctcaccaaaagttgaatcatctgtactaaaccactgcttttttatccagactttttatataaatcttttattttccaaaaaactgatcttttacctacccctcttagagttaaaaatattgcctgtcaggcaagagtatagtatgccaatataaataatatgctttatttggttagaaacagttggtttgggaagctagcaacatagcatattctttacaaatttaataaggtgtattttgatactgtgataacctgcattgtaaattaccaaatggttggaattgaccagtttatacttattaaaatttttgatgtgccaatggctatccaattcattgcatttgtgaattgtgcttttagaaaaattgtggacattttagttttatatacatatttatgagttatttgtgcatatgataaaattatatataataataaaagtatatatgtaacttacattgtgcccttgattattgaaaacttcctttttataacagattcactgtttggaagctaaagtaaaaatgagccatgttaccagaagtaataatttctatcttattactgatgtttttatactttgtggtaaaactatggaaagttaggttttcagatgctgtggtagctgaaagagtttgatgtacatgtggttaaagtgtgaagaaaatatgaaggaaaaagtatgaaaagtaccctagtcattacctaattgctattttgtttttaaggatctaagaagtgttattgcattgtacagattattttagaaattcacatctttgctggcttttcctttaacaccaagaatatctgttatcatctgtttggtactgtgttttgtttcctcttttaaagtaaaatattgaagtgatatttaaatgtttgcaagtctcatgaccttcctatagaaattcacattagtataataatttacattacaaatacaatatagcctttaattttgaagagtaaaaatggaaatggaagatgaattactatagtgtagttcacttaaatcgaaaatgtatatttgaatagtttcagtgaaatttggctcatatgaccatagtttaatagaattcttatttctattattgataaccttgaataaaaggatctaattataagttatctaggttttttcccttttagggaagagatgttatgtttttgtactactcttggctatagctgtaaaggatgtgtctgaacctggtaaaactttttaaaattctgagttcagttctgtaatattaatgaatattacattataaagatcacttaggaggggtttaatatatgctgatttgttttatatgaattgttagaaatatatacagaaataagggtagtttcaggctacctttcaggctattattagttgggcaagcttatttttagagcttttccctttcattggttggatgtagggcctgggaatacaaatagattttaatagttttactaggtaaaactgctagagagaaaattcatgtcccaagtagaaaaattaatatagctgaatacttaagtccttgttgaaaagttttctgaaatactggagttcattttcctgccttggtaaggcatttttaaaatttagtttagatggcttaaaccatttaaagaagctgtcttcattgtaaatatcaattgtcaatatcaattttcactgttcagaactgtccaaatactcttaaggtttgtctatactaaattcctattctttttaaaatttacctgttttccttctccctagtcccctttcctgccctttaaatctgaataaccagaagccatatattcaatgttttatgtattttcaatgttttgtgtataacgatatatgaagttagtgaattctgtaagacaaaaagatcgtttttattcacttttgattacaaaaaaaggttacatgaataaaataacaatttcctttaagagagggattcctgaatgattaaactgccaaggaaaaaagagtgaattcttccttttaataaaggtgacctaggtcctgaggaagttaggaaaaaagaaaaactcacattatacttgttaaatttgttttcaaatgtgattattaagttgttgtatttattttttgttatagacaaagcaaacccaaaaactagtctaaaaaagaattcctatgcattattaaaagagatagtaataaaatatgtattggtggtgaagaattccacaagcactcaagattgacataacctttaacaaagtggaaaaacttttattagaactgccaattctaggttcaaatttatgtcaaagcactttatggtaccataattagtacaactaaattattttttagctttaaatgtcatttttcactaaatgattttaaataagacatctgagagttacttgaggcaagtttagatacctgtacaagtttagattttgagaaactccctatttcctcattgtgtgtctctttcacatgctttttagaatcatttattccacaacatgtttccaaattctatctagtaatttttaaacttcaaaaataatctccctgttcaattacaaggttctaaagacaataaaataccttataatttcagtaacaacatttttctttttcttgggcaaagtattacaaagtgttcgcctaatcctcataatgttcttttaaattaacgtggaaatcagtaattatcctccttaaaaggtgggaaaactgaagcactgtaaagttaggttctgacccaaggtcagagtaaccaaggtgaaaaatctgggtatttcaacaactgctgttccagtgtatgtctattattattcgtatcaccttgaataaaatatggcatttaaaaatttatgatgtcataatgctgagtgagtctctactgagcagggctgcataatgttaaattttaaaaagaaaaattacaagcccggctttaaataataaagggattaagtacagaatatatatatttttaagatcatcgatgccattgtgtccaataaattgccttactaacagtgttatgttgtcttaagacagtgctgattagaaaaagtgtacaaagaatgctctaaagacccatggaacacaatataccttaaattggcactaagctataccacaataaaagtcatacatattgaatgttgacatacactgagaagggtgacgagttttcaataacgtattttagaaaattgttcattttttgcttaaatttatccgaatataagacctataaagcaagacaaggaagcatggagcactgagtcttttcatgcccagtatccaacagtcagagctatgttttcctcctgttcatgatggcttggcttttcagatggtgccaatcctgtgatgaggcacttgaagagtttgaaggttagggcatgtaaaatatggagctggaaggaagcatgctgctattccattggaagcaaaagggagtgtaggcccatagaatacttcttctttgccttctctgcttacatccagtacctggatacaagccagaggctcatttgtccaaattgaatatccaccaactaaatatattctcccattatggacagcaactccagattcattttggccagtcagcaggttgaaattacaacgtgtccactggtcagtgtctatgttgtaagaatctatatggcgcacaaggatccggtcattattgtagtctaggtcattgcctccaagaacataaagcttcctttgtacagcagccatggaatggtagacccttctctgcagcatggggctacggcttatccacttattctggttaggttcatacaccattagcctgttctgatattgtgccgtattagttactccacctgatatccaaagaagaccatcagccacatatccagcatggcatgaaagggatctgtcaaaggactgaacaaaagtccatttgttcttcttggggcaatatcgctcaactgtaggcagaacctggcgcagttcatttctgcccccaactgcatagaggtattcctccatggcacccagcacaaaatgctcccggcagtttttcatgggtgctatctctgcccaggaattactgcgggggtcatagcgacaggcagtcctcacagcacacgtccggccactggcatgctcaacttcccctcctgccacaaacaggaagtcccccatgactgccacacaatggtggctccttcccacaggcatgggagccagctcactccagttggcaatggcagctatgagagcattctcctgatcaacaggattgaagtaccgaagttccttgaccttgcagacctcgcgctttttcccaccaatgatatacagagtgtctgactggaatcgtggtttggtcctgcgagtctgccagacaggctgtgcatagatgctctggtggtattccagggcctcgttgacaagggctgttgcagtctcacttgcttggacaagggggtgggacagggcaactgtatggagagtatccacatccattaggccaaagcggatgtattgcaggagctcgtccatgtactggtagtggcagttgtgttccaaccacctcacagctagctgccagatctgctcttcactcagggaggtcaggcggtcgctcttcagcacctcctgaagcaggcaatagggaagcgttagaacttcttctgggcggctcttcaggagttcagagagatgtttcactaagaaatcgatcactgccttctccaacaaagtgaggttaaagaggtcagcaagtctgtacagatccaagtaattaaagctatttaattcctggatgagatagtgggagcataaattgagaagctccaacagctgtaggtgactgcccgctgctagcacatcctggatcacacctggctccagcaaaatctgtcctgtgtatgcaaactccagagcctgctttaagccaaggctggtcacaccgtgcaaattaacctcatcagctccactttccaccatacaaagactgaacattgcctttttatactgtcaggaattgttcacttcaaaattccatcaaatatggtgaaaacagatgagtacaatctggaaataaat

SEQ ID NO: 11327 - RNA, 6538 nt, Homo sapiens
  source 1..6538: mol_type = other RNA
ctgaatagctgggactacaggtgcccgccaccacgcccggctaattttttttgtatttttagtagagacggggtttcaccatgttgggctcgatctcctgacctcatgatccgcccgcctcggcctcccaaagtgctgggattacaggcgtgatgagccacctagtgctaattcatctctaaacctctgtagttggagtctcctgaaatctcagactacctcctgctttcattttctacccagggaatacactattgtcctaagttatttagccttgaaatgtcagaggcattttaggttcttcatgtttctcccactttcagttgattaccattacaggatcttaggcttctttttatctttttgcagtgccttgcatccactggttgtttgttttttctgttgggcactacttatttccttacctctggtttcttctcctacagcttatgttctgaaatgtgtattcctaaaatactgttttcctcttgttacttttctgctcgaggacttccagtaacttaccattgtttataaggtgatgttcaaacccttcagtctggagactttctgccacctatctgactgtacctttatcttcaagcttatctctttccaaacaagaggctcatttagcagctttctctgattgccatgttcatcctacactcagcctcattcagtttacagcatggaaactgtataggacctctttcctatagaaattgaagacacttaaataggaagaaaattaaaatatacatttggatacatgagtattccagtcaaataatatctataaaataccagatagagtataaaagacaactgaaggacaacagagtgatgaaaggactttattaggcatttggatttggttatgatttaaatttcaatttaattagaacgtttccatggcaaggaaggaagcatggaggactgtggaaaagtcattcagtattgagttcatttgcattagaggaatttcatagtttaaaacttgtatatctttacctatccttcgtatgttttcttcttaagcatatttgactttttctacctcagcatctgtataagaaaatatttgtgagtcagatgtttgtgggttttccttacctattattattttcttccatgctttacaacacattttttaaactaccttgttcttaaataattacacggacctgcttctgtgtactttcacagaatctttgacagttaaaaattgtatgttatataaaaatttgacaagcttctacagttaggaaaagcctttagaaatctgccttccccaaaccgtatgttatcatagcactcatgtctccccatgtctaaaaggtaaatagatacagaaacctcaccaaaagttgaatcatctgtactaaaccactgcttttttatccagactttttatataaatcttttattttccaaaaaactgatcttttacctacccctcttagagttaaaaatattgcctgtcaggcaagagtatagtatgccaatataaataatatgctttatttggttagaaacagttggtttgggaagctagcaacatagcatattctttacaaatttaataaggtgtattttgatactgtgataacctgcattgtaaattaccaaatggttggaattgaccagtttatacttattaaaatttttgatgtgccaatggctatccaattcattgcatttgtgaattgtgcttttagaaaaattgtggacattttagttttatatacatatttatgagttatttgtgcatatgataaaattatatataataataaaagtatatatgtaacttacattgtgcccttgattattgaaaacttcctttttataacagattcactgtttggaagctaaagtaaaaatgagccatgttaccagaagtaataatttctatcttattactgatgtttttatactttgtggtaaaactatggaaagttaggttttcagatgctgtggtagctgaaagagtttgatgtacatgtggttaaagtgtgaagaaaatatgaaggaaaaagtatgaaaagtaccctagtcattacctaattgctattttgtttttaaggatctaagaagtgttattgcattgtacagattattttagaaattcacatctttgctggcttttcctttaacaccaagaatatctgttatcatctgtttggtactgtgttttgtttcctcttttaaagtaaaatattgaagtgatatttaaatgtttgcaagtctcatgaccttcctatagaaattcacattagtataataatttacattacaaatacaatatagcctttaattttgaagagtaaaaatggaaatggaagatgaattactatagtgtagttcacttaaatcgaaaatgtatatttgaatagtttcagtgaaatttggctcatatgaccatagtttaatagaattcttatttctattattgataaccttgaataaaaggatctaattataagttatctaggttttttcccttttagggaagagatgttatgtttttgtactactcttggctatagctgtaaaggatgtgtctgaacctggtaaaactttttaaaattctgagttcagttctgtaatattaatgaatattacattataaagatcacttaggaggggtttaatatatgctgatttgttttatatgaattgttagaaatatatacagaaataagggtagtttcaggctacctttcaggctattattagttgggcaagcttatttttagagcttttccctttcattggttggatgtagggcctgggaatacaaatagattttaatagttttactaggtaaaactgctagagagaaaattcatgtcccaagtagaaaaattaatatagctgaatacttaagtccttgttgaaaagttttctgaaatactggagttcattttcctgccttggtaaggcatttttaaaatttagtttagatggcttaaaccatttaaagaagctgtcttcattgtaaatatcaattgtcaatatcaattttcactgttcagaactgtccaaatactcttaaggtttgtctatactaaattcctattctttttaaaatttacctgttttccttctccctagtcccctttcctgccctttaaatctgaataaccagaagccatatattcaatgttttatgtattttcaatgttttgtgtataacgatatatgaagttagtgaattctgtaagacaaaaagatcgtttttattcacttttgattacaaaaaaaggttacatgaataaaataacaatttcctttaagagagggattcctgaatgattaaactgccaaggaaaaaagagtgaattcttccttttaataaaggtgacctaggtcctgaggaagttaggaaaaaagaaaaactcacattatacttgttaaatttgttttcaaatgtgattattaagttgttgtatttattttttgttatagacaaagcaaacccaaaaactagtctaaaaaagaattcctatgcattattaaaagagatagtaataaaatatgtattggtggtgaagaattccacaagcactcaagattgacataacctttaacaaagtggaaaaacttttattagaactgccaattctaggttcaaatttatgtcaaagcactttatggtaccataattagtacaactaaattattttttagctttaaatgtcatttttcactaaatgattttaaataagacatctgagagttacttgaggcaagtttagatacctgtacaagtttagattttgagaaactccctatttcctcattgtgtgtctctttcacatgctttttagaatcatttattccacaacatgtttccaaattctatctagtaatttttaaacttcaaaaataatctccctgttcaattacaaggttctaaagacaataaaataccttataatttcagtaacaacatttttctttttcttgggcaaagtattacaaagtgttcgcctaatcctcataatgttcttttaaattaacgtggaaatcagtaattatcctccttaaaaggtgggaaaactgaagcactgtaaagttaggttctgacccaaggtcagagtaaccaaggtgaaaaatctgggtatttcaacaactgctgttccagtgtatgtctattattattcgtatcaccttgaataaaatatggcatttaaaaatttatgatgtcataatgctgagtgagtctctactgagcagggctgcataatgttaaattttaaaaagaaaaattacaagcccggctttaaataataaagggattaagtacagaatatatatatttttaagatcatcgatgccattgtgtccaataaattgccttactaacagtgttatgttgtcttaagacagtgctgattagaaaaagtgtacaaagaatgctctaaagacccatggaacacaatataccttaaattggcactaagctataccacaataaaagtcatacatattgaatgttgacatacactgagaagggtgacgagttttcaataacgtattttagaaaattgttcattttttgcttaaatttatccgaatataagacctataaagcaagacaaggaagcatggagcactgagtcttttcatgcccagtatccaacagtcagagctatgttttcctcctgttcatgatggcttggcttttcagatggtgccaatcctgtgatgaggcacttgaagagtttgaaggttagggcatgtaaaatatggagctggaaggaagcatgctgctattccattggaagcaaaagggagtgtaggcccatagaatacttcttctttgccttctctgcttacatccagtacttccattgtgcaagtgatcaaatgaagggtcccaaagccatttaaaaaacagtgttccagcactatagagaactgttgcccagttctgagttctaccaattctggatacaagccagaggctcatttgtccaaattgaatatccaccaactaaatatattctcccattatggacagcaactccagattcattttggccagtcagcaggttgaaattacaacgtgtccactggtcagtgtctatgttgtaagaatctatatggcgcacaaggatccggtcattattgtagtctaggtcattgcctccaagaacataaagcttcctttgtacagcagccatggaatggtagacccttctctgcagcatggggctacggcttatccacttattctggttaggttcatacaccattagcctgttctgatattgtgccgtattagttactccacctgatatccaaagaagaccatcagccacatatccagcatggcatgaaagggatctgtcaaaggactgaacaaaagtccatttgttcttcttggggcaatatcgctcaactgtaggcagaacctggcgcagttcatttctgcccccaactgcatagaggtattcctccatggcacccagcacaaaatgctcccggcagtttttcatgggtgctatctctgcccaggaattactgcgggggtcatagcgacaggcagtcctcacagcacacgtccggccactggcatgctcaacttcccctcctgccacaaacaggaagtcccccatgactgccacacaatggtggctccttcccacaggcatgggagccagctcactccagttggcaatggcagctatgagagcattctcctgatcaacaggattgaagtaccgaagttccttgaccttgcagacctcgcgctttttcccaccaatgatatacagagtgtctgactggaatcgtggtttggtcctgcgagtctgccagacaggctgtgcatagatgctctggtggtattccagggcctcgttgacaagggctgttgcagtctcacttgcttggacaagggggtgggacagggcaactgtatggagagtatccacatccattaggccaaagcggatgtattgcaggagctcgtccatgtactggtagtggcagttgtgttccaaccacctcacagctagctgccagatctgctcttcactcagggaggtcaggcggtcgctcttcagcacctcctgaagcaggcaatagggaagcgttagaacttcttctgggcggctcttcaggagttcagagagatgtttcactaagaaatcgatcactgccttctccaacaaagtgaggttaaagaggtcagcaagtctgtacagatccaagtaattaaagctatttaattcctggatgagatagtgggagcataaattgagaagctccaacagctgtaggtgactgcccgctgctagcacatcctggatcacacctggctccagcaaaatctgtcctgtgtatgcaaactccagagcctgctttaagccaaggctggtcacaccgtgcaaattaacctcatcagctccactttccaccatacaaagactgaacattgcctttttatactgtcaggaattgttcacttcaaaattccatcaaatatggtgaaaacagatgagtacaatctggaaataaatta

SEQ ID NO: 11328 - RNA, 4180 nt, Homo sapiens
  source 1..4180: mol_type = other RNA
ctgaatagctgggactacaggtgcccgccaccacgcctgactaatttttgtatttttagtagagacggggtttcaccatgttggccaggatggtcttgatctcctgaccttgtgatccgcctgcctcggcctcccaaagtgctgggattacaggtgcaagccaccgtgcctggcccaattttaaggtttctaaaagctagttgtagatattttaaaattggtaataacaataataatcagcaatagccctaattaaaaatttttggtcttcttgccaaaattaatatcttataaatgttaggatgatcataaagactgtttaacaagatggaaccagccccatgatggataagaggcgtgattccaatttttaaaatgctattagtgcaataatttattttaaattattctttgtacctcacaaaaacagcaagttattagaagaaagtataccagattagaagtaaggagatttggattccagctttagtcctattccctactaggctcgtcatctattgcaaatcactttaaattcctgagctttggtttctttatttacatcatttacttcatttagctccactgctaggctgtaaaaaacatgtagtattcgtgactgttcaccgctgtatctgcagtctcattcccaaggcagagcaggcactcagctaatgtttgctggctgaccgaattaaggattagaaactaaaaaatacaaatattgtcatgcattcttcagaaggttgccatgaggcctaagtgttatagtgaaatactatatgggaaaatgggtgcattcttttaaaattttttaaatgtggatacattcttggtacctaacttaaaagaaattaaggtaaatgggttaataattataagttattttaaatcactacgtttatatatgtgtaagtattttgcgaaaaacagactcagccaggtgcggtggctcatgcctgtagtcctagcactttgggaggccaaggtgggcagatcacttgagcccaggagttggagaccagcctgggcaacacagcaagagcccatctctacaaaaaatacagtaactagccagacgtggtggtgcacacctgtagtcccagctacttggaaggctgaggtgagaagatcacctgagcctgggaggtcaaggctgcagtgagctgtgatggtgctgctgcactccagcctgggtgtcagagtgagaccttgtctccaaaaaataaaaataaaaataagtaaaaagaaaaataggctctatttatctaaaggctctgaagacttcagttattgcttacgattaggaaggctttggagagaaaataacttgtgattttaatactgcaggtaaattctctaacacattcagattaaaaagtcaaatgttaattccctatgctacagcacagtcataatatgtaataccttaaccatattttgacaagataagagattgatgccactaaccttgaaagatctaagacattctcttaagtgaaaaataaaatatgtaaataatgtttatatttatataaagaaaatcaagctatatatttctagattttcaaatacatttgtataggaatacctcaaaaaaggcctagatagctcatacctgataacagtgatctacctttgaggaggggagtgagactgtatgagggcaaacagggacttttgctttattggcattgcctgaaattttttcatagtaggaatgtgaaaaaatagatgagagcatatactaatccactgaattccttaagccttacttgaatattgaagatggtccttgcaggaagggagcactgtggctttcagtagcacaacgtttaggcattctctctcttttttttcttttttttttgagacggagttttgctcttgttgcccaggctggagtgcaatggtgcaaacttggctcaccgcaacctccgccccaggttcaagtgattctcctgcctcagcctcccaagtagctaggattacaggcatgcgccaccatgcctggctaattttgtatttttagcagagatggggtttctccttgttggtctggctggtctcaaactcccgacctcaggggatctgccagcctcagcctcccaaagtgctgggattacaggtgtgagccaccacgcctggctaggcattcactcttacagtaggtgaaatagttttcctatagagaagaaaagctatatggctgacagcactgatattgaacattaaatatcatacttactaaaaaaaactaacccgcaaaattagaagggctaaggaaaaatatatttgctggttacatataatggtaatagaaagctagtaattaaatataattctcattagaattacaatatagcctttgaatattctattaaataaatgaattcaatttaagtttcattctcaaattaattttatcacatttgattggcccagtccattacacaaaaagacatactgactaaatacaacataatttctataacctgaggggactcgcacatcattacctgattgcttgctgacttggctgttgattggtttcatgactttgaagcttccctcctatgacaattcttcctcccctaaggacttcctcattgctgtttcttcatcttgccctaagagttctctctcttccataaacttcctttcctgggatgaccttctgtcatatgttgttctttgtaggtagcctccatctaaaagcagctcccgtgtctgtgacatgctctgctccaggaattcagaggcctccagtgactctgtcattgctccaggaccaccaggctcatcctcgggttctggagactgatgtgtgtcttccccatgctcatacatacacagcctcttttcaaccacctcacggatcaacatgtcaagcactgttcttcccaccatgctatattccatggttttttcaacttcattcattagccatggaagaaatcctatctcaatatctctttcaatgggatcataaaagtagccactatccctgaggctgccaaaaacagacgggagaaggtcagccaggtaacgctgtgcaaatgctcgggcggcgattttttgtgatgtctcgttgtgcttgtgcattatttcccactgctgtttcttacgccgttctttttcttctcggtgtcgcctctcttgctcttcaagtcgttgaacttcagcacgttcactattccgtagttcttcatactcacgctgactggcccgcaggttagccagctcttcttcttccattacttccagaagagactgctcaattgtcttccccaccaaaacttctaacactggtttaacttcaagatcaaagtcaaagagcagtggccctgtctggagtgcataagtgttacctcgaattacccttctgtcatacattatgtttccataatgcataggttcttcatctggctgcgtcaggctgtcccggtaacggctgcgctggcagggcagtgctcggggccggctggtgtaggtgtaggtgctcggggcccgagaggtgcgatcagtcagcgctgaggccatgtccgggggctgactgcctcgctttcggtggagcttggctttgaagcaggtgggcgctaaggtgttgtgggacccggagagatgtaagtagtgccaagggcaaggattccgcgacgcgaggagaggcgacaacaagggaggcgggcgggacgggaggttaccagcgcaggaggtgggagctatactgggctcgctcccagcaccacagagaccagctgcgggggccgcatcggttgcccagcaacccagggttctgtctgggggcgggaactccgggcagttccggtccccaggtttcccgggaaggactgcggcacaagggacttccggctcttgactccgcccagccgcgccacccaggtaggtgcgcctgcgctttgcgaggttcctggctagggaggcggccttggctggcttgaccgtcatccttgaggcctgcggggcaacggtggctgtccttggcccggctttggaatgtggctttgcagggctggtgttggcgccattctcgcaggcccacgtgctcctgctcttccagggtgtcctcggctgtttctcctgccgcggcgcagcagcgctcccaggctgcccccgcgataacacgcccctggcagccaggctcccagctctgttacgt

SEQ ID NO: 11329 - RNA, 3913 nt, Homo sapiens
  source 1..3913: mol_type = other RNA
ctgaatagctgggactacaggtgcccgccaccacgcctgactaatttttgtatttttagtagagacggggtttcaccatgttggccaggatggtcttgatctcctgaccttgtgatccgcctgcctcggcctcccaaagtgctgggattacaggtgcaagccaccgtgcctggcccaattttaaggtttctaaaagctagttgtagatattttaaaattggtaataacaataataatcagcaatagccctaattaaaaatttttggtcttcttgccaaaattaatatcttataaatgttaggatgatcataaagactgtttaacaagatggaaccagccccatgatggataagaggcgtgattccaatttttaaaatgctattagtgcaataatttattttaaattattctttgtacctcacaaaaacagcaagttattagaagaaagtataccagattagaagtaaggagatttggattccagctttagtcctattccctactaggctcgtcatctattgcaaatcactttaaattcctgagctttggtttctttatttacatcatttacttcatttagctccactgctaggctgtaaaaaacatgtagtattcgtgactgttcaccgctgtatctgcagtctcattcccaaggcagagcaggcactcagctaatgtttgctggctgaccgaattaaggattagaaactaaaaaatacaaatattgtcatgcattcttcagaaggttgccatgaggcctaagtgttatagtgaaatactatatgggaaaatgggtgcattcttttaaaattttttaaatgtggatacattcttggtacctaacttaaaagaaattaaggtaaatgggttaataattataagttattttaaatcactacgtttatatatgtgtaagtattttgcgaaaaacagactcagccaggtgcggtggctcatgcctgtagtcctagcactttgggaggccaaggtgggcagatcacttgagcccaggagttggagaccagcctgggcaacacagcaagagcccatctctacaaaaaatacagtaactagccagacgtggtggtgcacacctgtagtcccagctacttggaaggctgaggtgagaagatcacctgagcctgggaggtcaaggctgcagtgagctgtgatggtgctgctgcactccagcctgggtgtcagagtgagaccttgtctccaaaaaataaaaataaaaataagtaaaaagaaaaataggctctatttatctaaaggctctgaagacttcagttattgcttacgattaggaaggctttggagagaaaataacttgtgattttaatactgcaggtaaattctctaacacattcagattaaaaagtcaaatgttaattccctatgctacagcacagtcataatatgtaataccttaaccatattttgacaagataagagattgatgccactaaccttgaaagatctaagacattctcttaagtgaaaaataaaatatgtaaataatgtttatatttatataaagaaaatcaagctatatatttctagattttcaaatacatttgtataggaatacctcaaaaaaggcctagatagctcatacctgataacagtgatctacctttgaggaggggagtgagactgtatgagggcaaacagggacttttgctttattggcattgcctgaaattttttcatagtaggaatgtgaaaaaatagatgagagcatatactaatccactgaattccttaagccttacttgaatattgaagatggtccttgcaggaagggagcactgtggctttcagtagcacaacgtttaggcattctctctcttttttttcttttttttttgagacggagttttgctcttgttgcccaggctggagtgcaatggtgcaaacttggctcaccgcaacctccgccccaggttcaagtgattctcctgcctcagcctcccaagtagctaggattacaggcatgcgccaccatgcctggctaattttgtatttttagcagagatggggtttctccttgttggtctggctggtctcaaactcccgacctcaggggatctgccagcctcagcctcccaaagtgctgggattacaggtgtgagccaccacgcctggctaggcattcactcttacagtaggtgaaatagttttcctatagagaagaaaagctatatggctgacagcactgatattgaacattaaatatcatacttactaaaaaaaactaacccgcaaaattagaagggctaaggaaaaatatatttgctggttacatataatggtaatagaaagctagtaattaaatataattctcattagaattacaatatagcctttgaatattctattaaataaatgaattcaatttaagtttcattctcaaattaattttatcacatttgattggcccagtccattacacaaaaagacatactgactaaatacaacataatttctataacctgaggggactcgcacatcattacctgattgcttgctgacttggctgttgattggtttcatgactttgaagcttccctcctatgacaattcttcctcccctaaggacttcctcattgctgtttcttcatcttgccctaagagttctctctcttccataaacttcctttcctgggatgaccttctgtcatatgttgttctttgtaggtagcctccatctaaaagcagctcccgtgtctgtgacatgctctgctccaggaattcagaggcctccagtgactctgtcattgctccaggaccaccaggctcatcctcgggttctggagactgatgtgtgtcttccccatgctcatacatacacagcctcttttcaaccacctcacggatcaacatgtcaagcactgttcttcccaccatgctatattccatggttttttcaacttcattcattagccatggaagaaatcctatctcaatatctctttcaatgggatcataaaagtagccactatccctgaggctgccaaaaacagacgggagaaggtcagccaggtaacgctgtgcaaatgctcgggcggcgattttttgtgatgtctcgttgtgcttgtgcattatttcccactgctgtttcttacgccgttctttttcttctcggtgtcgcctctcttgctcttcaagtcgttgaacttcagcacgttcactattccgtagttcttcatactcacgctgactggcccgcaggttagccagctcttcttcttccattacttccagaagagactgctcaattgtcttccccaccaaaacttctaacactggtttaacttcaagatcaaagtcaaagagctctccttctagtatttgggtggccacatctttgccagttttggcaggaataaagagtggtgttggtggtctgtccaaaaatgcatctgtttggcattccatatcaacttctattatgcgatcagcaatttcttcaaggtataattcagtggccctgtctggagtgcataagtgttacctcgaattacccttctgtcatacattatgtttccataatgcataggttcttcatctggctgcgtcaggctgtcccggtaacggctgcgctggcagggcagtgctcggggccggctggtgtaggtgtaggtgctcggggcccgagaggtgcgatcagtcagcgctgaggccatgtccgggggctgactgcctcgctttcggtggagcttggctttgaagcaggtgggcgctaaggtgttgtgggacccggagagatgtaagtagtgccaagggcaaggattccgcgacgcgaggagaggcgacaacaagggaggcgggcgggacgggaggttaccagcgcaggaggtgggagctatactgggctcgctcccagcaccacagagaccagctgcggggg

SEQ ID NO: 11330 - RNA, 4483 nt, Homo sapiens
  source 1..4483: mol_type = other RNA
ctgaatagctgggactacaggtgcccgccaccacgcctgactaatttttgtatttttagtagagacggggtttcaccatgttggccaggatggtcttgatctcctgaccttgtgatccgcctgcctcggcctcccaaagtgctgggattacaggtgcaagccaccgtgcctggcccaattttaaggtttctaaaagctagttgtagatattttaaaattggtaataacaataataatcagcaatagccctaattaaaaatttttggtcttcttgccaaaattaatatcttataaatgttaggatgatcataaagactgtttaacaagatggaaccagccccatgatggataagaggcgtgattccaatttttaaaatgctattagtgcaataatttattttaaattattctttgtacctcacaaaaacagcaagttattagaagaaagtataccagattagaagtaaggagatttggattccagctttagtcctattccctactaggctcgtcatctattgcaaatcactttaaattcctgagctttggtttctttatttacatcatttacttcatttagctccactgctaggctgtaaaaaacatgtagtattcgtgactgttcaccgctgtatctgcagtctcattcccaaggcagagcaggcactcagctaatgtttgctggctgaccgaattaaggattagaaactaaaaaatacaaatattgtcatgcattcttcagaaggttgccatgaggcctaagtgttatagtgaaatactatatgggaaaatgggtgcattcttttaaaattttttaaatgtggatacattcttggtacctaacttaaaagaaattaaggtaaatgggttaataattataagttattttaaatcactacgtttatatatgtgtaagtattttgcgaaaaacagactcagccaggtgcggtggctcatgcctgtagtcctagcactttgggaggccaaggtgggcagatcacttgagcccaggagttggagaccagcctgggcaacacagcaagagcccatctctacaaaaaatacagtaactagccagacgtggtggtgcacacctgtagtcccagctacttggaaggctgaggtgagaagatcacctgagcctgggaggtcaaggctgcagtgagctgtgatggtgctgctgcactccagcctgggtgtcagagtgagaccttgtctccaaaaaataaaaataaaaataagtaaaaagaaaaataggctctatttatctaaaggctctgaagacttcagttattgcttacgattaggaaggctttggagagaaaataacttgtgattttaatactgcaggtaaattctctaacacattcagattaaaaagtcaaatgttaattccctatgctacagcacagtcataatatgtaataccttaaccatattttgacaagataagagattgatgccactaaccttgaaagatctaagacattctcttaagtgaaaaataaaatatgtaaataatgtttatatttatataaagaaaatcaagctatatatttctagattttcaaatacatttgtataggaatacctcaaaaaaggcctagatagctcatacctgataacagtgatctacctttgaggaggggagtgagactgtatgagggcaaacagggacttttgctttattggcattgcctgaaattttttcatagtaggaatgtgaaaaaatagatgagagcatatactaatccactgaattccttaagccttacttgaatattgaagatggtccttgcaggaagggagcactgtggctttcagtagcacaacgtttaggcattctctctcttttttttcttttttttttgagacggagttttgctcttgttgcccaggctggagtgcaatggtgcaaacttggctcaccgcaacctccgccccaggttcaagtgattctcctgcctcagcctcccaagtagctaggattacaggcatgcgccaccatgcctggctaattttgtatttttagcagagatggggtttctccttgttggtctggctggtctcaaactcccgacctcaggggatctgccagcctcagcctcccaaagtgctgggattacaggtgtgagccaccacgcctggctaggcattcactcttacagtaggtgaaatagttttcctatagagaagaaaagctatatggctgacagcactgatattgaacattaaatatcatacttactaaaaaaaactaacccgcaaaattagaagggctaaggaaaaatatatttgctggttacatataatggtaatagaaagctagtaattaaatataattctcattagaattacaatatagcctttgaatattctattaaataaatgaattcaatttaagtttcattctcaaattaattttatcacatttgattggcccagtccattacacaaaaagacatactgactaaatacaacataatttctataacctgaggggactcgcacatcattacctgattgcttgctgacttggctgttgattggtttcatgactttgaagcttccctcctatgacaattcttcctcccctaaggacttcctcattgctgtttcttcatcttgccctaagagttctctctcttccataaacttcctttcctgggatgaccttctgtcatatgttgttctttgtaggtagcctccatctaaaagcagctcccgtgtctgtgacatgctctgctccaggaattcagaggcctccagtgactctgtcattgctccaggaccaccaggctcatcctcgggttctggagactgatgtgtgtcttccccatgctcatacatacacagcctcttttcaaccacctcacggatcaacatgtcaagcactgttcttcccaccatgctatattccatggttttttcaacttcattcattagccatggaagaaatcctatctcaatatctctttcaatgggatcataaaagtagccactatccctgaggctgccaaaaacagacgggagaaggtcagccaggtaacgctgtgcaaatgctcgggcggcgattttttgtgatgtctcgttgtgcttgtgcattatttcccactgctgtttcttacgccgttctttttcttctcggtgtcgcctctcttgctcttcaagtcgttgaacttcagcacgttcactattccgtagttcttcatactcacgctgactggcccgcaggttagccagctcttcttcttccattacttccagaagagactgctcaattgtcttccccaccaaaacttctaacactggtttaacttcaagatcaaagtcaaagagctctccttctagtatttgggtggccacatctttgccagttttggcaggaataaagagtggtgttggtggtctgtccaaaaatgcatctgtttggcattccatatcaacttctattatgcgatcagcaatttcttcaaggtataattctgtttgcacatcgacatgctttctgccttccacaggttcaggtgtttgtggtctgagctgctcttgggcttgttttctggcaagagccctcttcctagcctcccgttgtctctggagctctagagaatcaggccgtccgagcagtggccctgtctggagtgcataagtgttacctcgaattacccttctgtcatacattatgtttccataatgcataggttcttcatctggctgcgtcaggctgtcccggtaacggctgcgctggcagggcagtgctcggggccggctggtgtaggtgtaggtgctcggggcccgagaggtgcgatcagtcagcgctgaggccatgtccgggggctgactgcctcgctttcggtggagcttggctttgaagcaggtgggcgctaaggtgttgtgggacccggagagatgtaagtagtgccaagggcaaggattccgcgacgcgaggagaggcgacaacaagggaggcgggcgggacgggaggttaccagcgcaggaggtgggagctatactgggctcgctcccagcaccacagagaccagctgcgggggccgcatcggttgcccagcaacccagggttctgtctgggggcgggaactccgggcagttccggtccccaggtttcccgggaaggactgcggcacaagggacttccggctcttgactccgcccagccgcgccacccaggtaggtgcgcctgcgctttgcgaggttcctggctagggaggcggccttggctggcttgaccgtcatccttgaggcctgcggggcaacggtggctgtccttggcccggctttggaatgtggctttgcagggctggtgttggcgccattctcgcaggcccacgtgctcctgctcttccagggtgtcctcggctgtttctcctgccgcggcgcagcagcgctcccaggctgcccccgcgataacacgcccctggcagccaggctcccagctctgttacgtgcccgggcggggaag

SEQ ID NO: 11331 - RNA, 4002 nt, Homo sapiens
  source 1..4002: mol_type = other RNA
ctgaatagctgggactacaggtgcccgccaccacgcctgactaatttttgtatttttagtagagacggggtttcaccatgttggccaggatggtcttgatctcctgaccttgtgatccgcctgcctcggcctcccaaagtgctgggattacaggtgcaagccaccgtgcctggcccaattttaaggtttctaaaagctagttgtagatattttaaaattggtaataacaataataatcagcaatagccctaattaaaaatttttggtcttcttgccaaaattaatatcttataaatgttaggatgatcataaagactgtttaacaagatggaaccagccccatgatggataagaggcgtgattccaatttttaaaatgctattagtgcaataatttattttaaattattctttgtacctcacaaaaacagcaagttattagaagaaagtataccagattagaagtaaggagatttggattccagctttagtcctattccctactaggctcgtcatctattgcaaatcactttaaattcctgagctttggtttctttatttacatcatttacttcatttagctccactgctaggctgtaaaaaacatgtagtattcgtgactgttcaccgctgtatctgcagtctcattcccaaggcagagcaggcactcagctaatgtttgctggctgaccgaattaaggattagaaactaaaaaatacaaatattgtcatgcattcttcagaaggttgccatgaggcctaagtgttatagtgaaatactatatgggaaaatgggtgcattcttttaaaattttttaaatgtggatacattcttggtacctaacttaaaagaaattaaggtaaatgggttaataattataagttattttaaatcactacgtttatatatgtgtaagtattttgcgaaaaacagactcagccaggtgcggtggctcatgcctgtagtcctagcactttgggaggccaaggtgggcagatcacttgagcccaggagttggagaccagcctgggcaacacagcaagagcccatctctacaaaaaatacagtaactagccagacgtggtggtgcacacctgtagtcccagctacttggaaggctgaggtgagaagatcacctgagcctgggaggtcaaggctgcagtgagctgtgatggtgctgctgcactccagcctgggtgtcagagtgagaccttgtctccaaaaaataaaaataaaaataagtaaaaagaaaaataggctctatttatctaaaggctctgaagacttcagttattgcttacgattaggaaggctttggagagaaaataacttgtgattttaatactgcaggtaaattctctaacacattcagattaaaaagtcaaatgttaattccctatgctacagcacagtcataatatgtaataccttaaccatattttgacaagataagagattgatgccactaaccttgaaagatctaagacattctcttaagtgaaaaataaaatatgtaaataatgtttatatttatataaagaaaatcaagctatatatttctagattttcaaatacatttgtataggaatacctcaaaaaaggcctagatagctcatacctgataacagtgatctacctttgaggaggggagtgagactgtatgagggcaaacagggacttttgctttattggcattgcctgaaattttttcatagtaggaatgtgaaaaaatagatgagagcatatactaatccactgaattccttaagccttacttgaatattgaagatggtccttgcaggaagggagcactgtggctttcagtagcacaacgtttaggcattctctctcttttttttcttttttttttgagacggagttttgctcttgttgcccaggctggagtgcaatggtgcaaacttggctcaccgcaacctccgccccaggttcaagtgattctcctgcctcagcctcccaagtagctaggattacaggcatgcgccaccatgcctggctaattttgtatttttagcagagatggggtttctccttgttggtctggctggtctcaaactcccgacctcaggggatctgccagcctcagcctcccaaagtgctgggattacaggtgtgagccaccacgcctggctaggcattcactcttacagtaggtgaaatagttttcctatagagaagaaaagctatatggctgacagcactgatattgaacattaaatatcatacttactaaaaaaaactaacccgcaaaattagaagggctaaggaaaaatatatttgctggttacatataatggtaatagaaagctagtaattaaatataattctcattagaattacaatatagcctttgaatattctattaaataaatgaattcaatttaagtttcattctcaaattaattttatcacatttgattggcccagtccattacacaaaaagacatactgactaaatacaacataatttctataacctgaggggactcgcacatcattacctgattgcttgctgacttggctgttgattggtttcatgactttgaagcttccctcctatgacaattcttcctcccctaaggacttcctcattgctgtttcttcatcttgccctaagagttctctctcttccataaacttcctttcctgggatgaccttctgtcatatgttgttctttgtaggtagcctccatctaaaagcagctcccgtgtctgtgacatgctctgctccaggaattcagaggcctccagtgactctgtcattgctccaggaccaccaggctcatcctcgggttctggagactgatgtgtgtcttccccatgctcatacatacacagcctcttttcaaccacctcacggatcaacatgtcaagcactgttcttcccaccatgctatattccatggttttttcaacttcattcattagccatggaagaaatcctatctcaatatctctttcaatgggatcataaaagtagccactatccctgaggctgccaaaaacagacgggagaaggtcagccaggtaacgctgtgcaaatgctcgggcggcgattttttgtgatgtctcgttgtgcttgtgcattatttcccactgctgtttcttacgccgttctttttcttctcggtgtcgcctctcttgctcttcaagtcgttgaacttcagcacgttcactattccgtagttcttcatactcacgctgactggcccgcaggttagccagctcttcttcttccattacttccagaagagactgctcaattgtcttccccaccaaaacttctaacactggtttaacttcaagatcaaagtcaaagagctctccttctagtatttgggtggccacatctttgccagttttggcaggaataaagagtggtgttggtggtctgtccaaaaatgcatctgtttggcattccatatcaacttctattatgcgatcagcaatttcttcaaggtataattctgtttgcacatcgacatgctttctgccttccacaggttcaggtgtttgtggtctgagctgctcttgggcttgttttctggcaagagccctcttcctagcctcccgttgtctctggagctctagagaatcaggccgtccgagggctgcgtcaggctgtcccggtaacggctgcgctggcagggcagtgctcggggccggctggtgtaggtgtaggtgctcggggcccgagaggtgcgatcagtcagcgctgaggccatgtccgggggctgactgcctcgctttcggtggagcttggctttgaagcaggtgggcgctaaggtgttgtgggacccggagagatgtaagtagtgccaagggcaaggattccgcgacgcgaggagaggcgacaacaagggaggcgggcgggacgggaggttaccagcgcaggaggtgggagctatactgggctcgctcccagcaccacagagaccagctgcgggggccgcatcggttgcccagcaacccagggttctgtct

SEQ ID NO: 11332 - RNA, 4085 nt, Homo sapiens
  source 1..4085: mol_type = other RNA
ctgaatagctgggactacaggtgcccgccaccacgcctgactaatttttgtatttttagtagagacggggtttcaccatgttggccaggatggtcttgatctcctgaccttgtgatccgcctgcctcggcctcccaaagtgctgggattacaggtgcaagccaccgtgcctggcccaattttaaggtttctaaaagctagttgtagatattttaaaattggtaataacaataataatcagcaatagccctaattaaaaatttttggtcttcttgccaaaattaatatcttataaatgttaggatgatcataaagactgtttaacaagatggaaccagccccatgatggataagaggcgtgattccaatttttaaaatgctattagtgcaataatttattttaaattattctttgtacctcacaaaaacagcaagttattagaagaaagtataccagattagaagtaaggagatttggattccagctttagtcctattccctactaggctcgtcatctattgcaaatcactttaaattcctgagctttggtttctttatttacatcatttacttcatttagctccactgctaggctgtaaaaaacatgtagtattcgtgactgttcaccgctgtatctgcagtctcattcccaaggcagagcaggcactcagctaatgtttgctggctgaccgaattaaggattagaaactaaaaaatacaaatattgtcatgcattcttcagaaggttgccatgaggcctaagtgttatagtgaaatactatatgggaaaatgggtgcattcttttaaaattttttaaatgtggatacattcttggtacctaacttaaaagaaattaaggtaaatgggttaataattataagttattttaaatcactacgtttatatatgtgtaagtattttgcgaaaaacagactcagccaggtgcggtggctcatgcctgtagtcctagcactttgggaggccaaggtgggcagatcacttgagcccaggagttggagaccagcctgggcaacacagcaagagcccatctctacaaaaaatacagtaactagccagacgtggtggtgcacacctgtagtcccagctacttggaaggctgaggtgagaagatcacctgagcctgggaggtcaaggctgcagtgagctgtgatggtgctgctgcactccagcctgggtgtcagagtgagaccttgtctccaaaaaataaaaataaaaataagtaaaaagaaaaataggctctatttatctaaaggctctgaagacttcagttattgcttacgattaggaaggctttggagagaaaataacttgtgattttaatactgcaggtaaattctctaacacattcagattaaaaagtcaaatgttaattccctatgctacagcacagtcataatatgtaataccttaaccatattttgacaagataagagattgatgccactaaccttgaaagatctaagacattctcttaagtgaaaaataaaatatgtaaataatgtttatatttatataaagaaaatcaagctatatatttctagattttcaaatacatttgtataggaatacctcaaaaaaggcctagatagctcatacctgataacagtgatctacctttgaggaggggagtgagactgtatgagggcaaacagggacttttgctttattggcattgcctgaaattttttcatagtaggaatgtgaaaaaatagatgagagcatatactaatccactgaattccttaagccttacttgaatattgaagatggtccttgcaggaagggagcactgtggctttcagtagcacaacgtttaggcattctctctcttttttttcttttttttttgagacggagttttgctcttgttgcccaggctggagtgcaatggtgcaaacttggctcaccgcaacctccgccccaggttcaagtgattctcctgcctcagcctcccaagtagctaggattacaggcatgcgccaccatgcctggctaattttgtatttttagcagagatggggtttctccttgttggtctggctggtctcaaactcccgacctcaggggatctgccagcctcagcctcccaaagtgctgggattacaggtgtgagccaccacgcctggctaggcattcactcttacagtaggtgaaatagttttcctgattgcttgctgacttggctgttgattggtttcatgactttgaagcttccctcctatgacaattcttcctcccctaaggacttcctcattgctgtttcttcatcttgccctaagagttctctctcttccataaacttcctttcctgggatgaccttctgtcatatgttgttctttgtaggtagcctccatctaaaagcagctcccgtgtctgtgacatgctctgctccaggaattcagaggcctccagtgactctgtcattgctccaggaccaccaggctcatcctcgggttctggagactgatgtgtgtcttccccatgctcatacatacacagcctcttttcaaccacctcacggatcaacatgtcaagcactgttcttcccaccatgctatattccatggttttttcaacttcattcattagccatggaagaaatcctatctcaatatctctttcaatgggatcataaaagtagccactatccctgaggctgccaaaaacagacgggagaaggtcagccaggtaacgctgtgcaaatgctcgggcggcgattttttgtgatgtctcgttgtgcttgtgcattatttcccactgctgtttcttacgccgttctttttcttctcggtgtcgcctctcttgctcttcaagtcgttgaacttcagcacgttcactattccgtagttcttcatactcacgctgactggcccgcaggttagccagctcttcttcttccattacttccagaagagactgctcaattgtcttccccaccaaaacttctaacactggtttaacttcaagatcaaagtcaaagagcagtggccctgtctggagtgcataagtgttacctcgaattacccttctgtcatacattatgtttccataatgcataggttcttcatctggctgcgtcaggctgtcccggtaacggctgcgctggcagggcagtgctcggggccggctggtgtaggtgtaggtgctcggggcccgagaggtgcgatcagtcagcgctgaggccatgtccgggggctgactgcctcgctttcggtggagcttggctttgaagcaggtgggcgctaaggtgttgtgggacccggagagatgtaagtagtgccaagggcaaggattccgcgacgcgaggagaggcgacaacaagggaggcgggcgggacgggaggttaccagcgcaggaggtgggagctatactgggctcgctcccagcaccacagagaccagctgcgggggccgcatcggttgcccagcaacccagggttctgtctgggggcgggaactccgggcagttccggtccccaggtttcccgggaaggactgcggcacaagggacttccggctcttgactccgcccagccgcgccacccaggtaggtgcgcctgcgctttgcgaggttcctggctagggaggcggccttggctggcttgaccgtcatccttgaggcctgcggggcaacggtggctgtccttggcccggctttggaatgtggctttgcagggctggtgttggcgccattctcgcaggcccacgtgctcctgctcttccagggtgtcctcggctgtttctcctgccgcggcgcagcagcgctcccaggctgcccccgcgataacacgcccctggcagccaggctcccagctctgttacgtgcccgggcggggaagagcttcctggtgtctcccggctcctgcccttctcccgccccaggggcgggctgccgccgccctctgcagctgagtcagtgcagttcctcacctaccttctctgctcaccgctgtgtgctagcaatcggaggacccttggcacacggagcgacaggggcctcccccacagacacctcattttgggaaagaagtgagcaatttattgagtcttaaaaaatacaaag

SEQ ID NO: 11333 - RNA, 3579 nt, Homo sapiens
  source 1..3579: mol_type = other RNA
ctgaatagctgggactacaggtgcccgccaccacgcctgactaatttttgtatttttagtagagacggggtttcaccatgttggccaggatggtcttgatctcctgaccttgtgatccgcctgcctcggcctcccaaagtgctgggattacaggtgcaagccaccgtgcctggcccaattttaaggtttctaaaagctagttgtagatattttaaaattggtaataacaataataatcagcaatagccctaattaaaaatttttggtcttcttgccaaaattaatatcttataaatgttaggatgatcataaagactgtttaacaagatggaaccagccccatgatggataagaggcgtgattccaatttttaaaatgctattagtgcaataatttattttaaattattctttgtacctcacaaaaacagcaagttattagaagaaagtataccagattagaagtaaggagatttggattccagctttagtcctattccctactaggctcgtcatctattgcaaatcactttaaattcctgagctttggtttctttatttacatcatttacttcatttagctccactgctaggctgtaaaaaacatgtagtattcgtgactgttcaccgctgtatctgcagtctcattcccaaggcagagcaggcactcagctaatgtttgctggctgaccgaattaaggattagaaactaaaaaatacaaatattgtcatgcattcttcagaaggttgccatgaggcctaagtgttatagtgaaatactatatgggaaaatgggtgcattcttttaaaattttttaaatgtggatacattcttggtacctaacttaaaagaaattaaggtaaatgggttaataattataagttattttaaatcactacgtttatatatgtgtaagtattttgcgaaaaacagactcagccaggtgcggtggctcatgcctgtagtcctagcactttgggaggccaaggtgggcagatcacttgagcccaggagttggagaccagcctgggcaacacagcaagagcccatctctacaaaaaatacagtaactagccagacgtggtggtgcacacctgtagtcccagctacttggaaggctgaggtgagaagatcacctgagcctgggaggtcaaggctgcagtgagctgtgatggtgctgctgcactccagcctgggtgtcagagtgagaccttgtctccaaaaaataaaaataaaaataagtaaaaagaaaaataggctctatttatctaaaggctctgaagacttcagttattgcttacgattaggaaggctttggagagaaaataacttgtgattttaatactgcaggtaaattctctaacacattcagattaaaaagtcaaatgttaattccctatgctacagcacagtcataatatgtaataccttaaccatattttgacaagataagagattgatgccactaaccttgaaagatctaagacattctcttaagtgaaaaataaaatatgtaaataatgtttatatttatataaagaaaatcaagctatatatttctagattttcaaatacatttgtataggaatacctcaaaaaaggcctagatagctcatacctgataacagtgatctacctttgaggaggggagtgagactgtatgagggcaaacagggacttttgctttattggcattgcctgaaattttttcatagtaggaatgtgaaaaaatagatgagagcatatactaatccactgaattccttaagccttacttgaatattgaagatggtccttgcaggaagggagcactgtggctttcagtagcacaacgtttaggcattctctctcttttttttcttttttttttgagacggagttttgctcttgttgcccaggctggagtgcaatggtgcaaacttggctcaccgcaacctccgccccaggttcaagtgattctcctgcctcagcctcccaagtagctaggattacaggcatgcgccaccatgcctggctaattttgtatttttagcagagatggggtttctccttgttggtctggctggtctcaaactcccgacctcaggggatctgccagcctcagcctcccaaagtgctgggattacaggtgtgagccaccacgcctggctaggcattcactcttacagtaggtgaaatagttttcctgattgcttgctgacttggctgttgattggtttcatgactttgaagcttccctcctatgacaattcttcctcccctaaggacttcctcattgctgtttcttcatcttgccctaagagttctctctcttccataaacttcctttcctgggatgaccttctgtcatatgttgttctttgtaggtagcctccatctaaaagcagctcccgtgtctgtgacatgctctgctccaggaattcagaggcctccagtgactctgtcattgctccaggaccaccaggctcatcctcgggttctggagactgatgtgtgtcttccccatgctcatacatacacagcctcttttcaaccacctcacggatcaacatgtcaagcactgttcttcccaccatgctatattccatggttttttcaacttcattcattagccatggaagaaatcctatctcaatatctctttcaatgggatcataaaagtagccactatccctgaggctgccaaaaacagacgggagaaggtcagccaggtaacgctgtgcaaatgctcgggcggcgattttttgtgatgtctcgttgtgcttgtgcattatttcccactgctgtttcttacgccgttctttttcttctcggtgtcgcctctcttgctcttcaagtcgttgaacttcagcacgttcactattccgtagttcttcatactcacgctgactggcccgcaggttagccagctcttcttcttccattacttccagaagagactgctcaattgtcttccccaccaaaacttctaacactggtttaacttcaagatcaaagtcaaagagctctccttctagtatttgggtggccacatctttgccagttttggcaggaataaagagtggtgttggtggtctgtccaaaaatgcatctgtttggcattccatatcaacttctattatgcgatcagcaatttcttcaaggtataattcagtggccctgtctggagtgcataagtgttacctcgaattacccttctgtcatacattatgtttccataatgcataggttcttcatctggctgcgtcaggctgtcccggtaacggctgcgctggcagggcagtgctcggggccggctggtgtaggtgtaggtgctcggggcccgagaggtgcgatcagtcagcgctgaggccatgtccgggggctgactgcctcgctttcggtggagcttggctttgaagcaggtgggcgctaaggtgttgtgggacccggagagatgtaagtagtgccaagggcaaggattccgcgacgcgaggagaggcgacaacaagggaggcgggcgggacgggaggttaccagcgcaggaggtgggagctatactgggctcgctcccagcaccacagagaccagctgcggggg

SEQ ID NO: 11334 - RNA, 4134 nt, Homo sapiens
  source 1..4134: mol_type = other RNA
ctgaatagctgggactacaggtgcccgccaccacgcctgactaatttttgtatttttagtagagacggggtttcaccatgttggccaggatggtcttgatctcctgaccttgtgatccgcctgcctcggcctcccaaagtgctgggattacaggtgcaagccaccgtgcctggcccaattttaaggtttctaaaagctagttgtagatattttaaaattggtaataacaataataatcagcaatagccctaattaaaaatttttggtcttcttgccaaaattaatatcttataaatgttaggatgatcataaagactgtttaacaagatggaaccagccccatgatggataagaggcgtgattccaatttttaaaatgctattagtgcaataatttattttaaattattctttgtacctcacaaaaacagcaagttattagaagaaagtataccagattagaagtaaggagatttggattccagctttagtcctattccctactaggctcgtcatctattgcaaatcactttaaattcctgagctttggtttctttatttacatcatttacttcatttagctccactgctaggctgtaaaaaacatgtagtattcgtgactgttcaccgctgtatctgcagtctcattcccaaggcagagcaggcactcagctaatgtttgctggctgaccgaattaaggattagaaactaaaaaatacaaatattgtcatgcattcttcagaaggttgccatgaggcctaagtgttatagtgaaatactatatgggaaaatgggtgcattcttttaaaattttttaaatgtggatacattcttggtacctaacttaaaagaaattaaggtaaatgggttaataattataagttattttaaatcactacgtttatatatgtgtaagtattttgcgaaaaacagactcagccaggtgcggtggctcatgcctgtagtcctagcactttgggaggccaaggtgggcagatcacttgagcccaggagttggagaccagcctgggcaacacagcaagagcccatctctacaaaaaatacagtaactagccagacgtggtggtgcacacctgtagtcccagctacttggaaggctgaggtgagaagatcacctgagcctgggaggtcaaggctgcagtgagctgtgatggtgctgctgcactccagcctgggtgtcagagtgagaccttgtctccaaaaaataaaaataaaaataagtaaaaagaaaaataggctctatttatctaaaggctctgaagacttcagttattgcttacgattaggaaggctttggagagaaaataacttgtgattttaatactgcaggtaaattctctaacacattcagattaaaaagtcaaatgttaattccctatgctacagcacagtcataatatgtaataccttaaccatattttgacaagataagagattgatgccactaaccttgaaagatctaagacattctcttaagtgaaaaataaaatatgtaaataatgtttatatttatataaagaaaatcaagctatatatttctagattttcaaatacatttgtataggaatacctcaaaaaaggcctagatagctcatacctgataacagtgatctacctttgaggaggggagtgagactgtatgagggcaaacagggacttttgctttattggcattgcctgaaattttttcatagtaggaatgtgaaaaaatagatgagagcatatactaatccactgaattccttaagccttacttgaatattgaagatggtccttgcaggaagggagcactgtggctttcagtagcacaacgtttaggcattctctctcttttttttcttttttttttgagacggagttttgctcttgttgcccaggctggagtgcaatggtgcaaacttggctcaccgcaacctccgccccaggttcaagtgattctcctgcctcagcctcccaagtagctaggattacaggcatgcgccaccatgcctggctaattttgtatttttagcagagatggggtttctccttgttggtctggctggtctcaaactcccgacctcaggggatctgccagcctcagcctcccaaagtgctgggattacaggtgtgagccaccacgcctggctaggcattcactcttacagtaggtgaaatagttttcctgattgcttgctgacttggctgttgattggtttcatgactttgaagcttccctcctatgacaattcttcctcccctaaggacttcctcattgctgtttcttcatcttgccctaagagttctctctcttccataaacttcctttcctgggatgaccttctgtcatatgttgttctttgtaggtagcctccatctaaaagcagctcccgtgtctgtgacatgctctgctccaggaattcagaggcctccagtgactctgtcattgctccaggaccaccaggctcatcctcgggttctggagactgatgtgtgtcttccccatgctcatacatacacagcctcttttcaaccacctcacggatcaacatgtcaagcactgttcttcccaccatgctatattccatggttttttcaacttcattcattagccatggaagaaatcctatctcaatatctctttcaatgggatcataaaagtagccactatccctgaggctgccaaaaacagacgggagaaggtcagccaggtaacgctgtgcaaatgctcgggcggcgattttttgtgatgtctcgttgtgcttgtgcattatttcccactgctgtttcttacgccgttctttttcttctcggtgtcgcctctcttgctcttcaagtcgttgaacttcagcacgttcactattccgtagttcttcatactcacgctgactggcccgcaggttagccagctcttcttcttccattacttccagaagagactgctcaattgtcttccccaccaaaacttctaacactggtttaacttcaagatcaaagtcaaagagctctccttctagtatttgggtggccacatctttgccagttttggcaggaataaagagtggtgttggtggtctgtccaaaaatgcatctgtttggcattccatatcaacttctattatgcgatcagcaatttcttcaaggtataattctgtttgcacatcgacatgctttctgccttccacaggttcaggtgtttgtggtctgagctgctcttgggcttgttttctggcaagagccctcttcctagcctcccgttgtctctggagctctagagaatcaggccgtccgagcagtggccctgtctggagtgcataagtgttacctcgaattacccttctgtcatacattatgtttccataatgcataggttcttcatctggctgcgtcaggctgtcccggtaacggctgcgctggcagggcagtgctcggggccggctggtgtaggtgtaggtgctcggggcccgagaggtgcgatcagtcagcgctgaggccatgtccgggggctgactgcctcgctttcggtggagcttggctttgaagcaggtgggcgctaaggtgttgtgggacccggagagatgtaagtagtgccaagggcaaggattccgcgacgcgaggagaggcgacaacaagggaggcgggcgggacgggaggttaccagcgcaggaggtgggagctatactgggctcgctcccagcaccacagagaccagctgcgggggccgcatcggttgcccagcaacccagggttctgtctgggggcgggaactccgggcagttccggtccccaggtttcccgggaaggactgcggcacaagggacttccggctcttgactccgcccagccgcgccacccaggtaggtgcgcctgcgctttgcgaggttcctggctagggaggcggccttggctggcttgaccgtcatccttgaggcctgcggggcaacggtggctgtccttggcccggctttggaatgtggctttgcagggctggtgttggcgccattctcgcaggcccacgtgctcctgctcttccagggtgtcctcggctgtttctcctgccgcggcgcagcagcgctcccaggctgcccccgcgataacacgcccctggcagccaggctcccagctctgttacgt

SEQ ID NO: 11335 - RNA, 7242 nt, Homo sapiens
  source 1..7242: mol_type = other RNA
ctgaatagctgggactacaggtgcccgccaccacgcctggctaattttttattttttgtatttttagtagagacagggtttcactatgttagccaggatggtctcgatctcctgacctcgtgatctgcctgccttggcctcccaaagtgctgggattacaggtgtgagccactgcgcccggccttttccttgacattttcaaagaactatgcatgtaatattatagtgactgttcacccagccccttgccctaaagcctggtaacatgattaactcatgattcctggataaatgctatgttctcattcctccatttttatctatacgtaaggctcttggctttgaattttatttctatctctttgtttggttaagttcatcttggtaaaacattagctctccccgcatttgttctcagttctatgatgtagagttgataaactttcccagtaggacagacacatattttgcccaatgtgtgttctctgtaaatgcaggtgaggaaggaggggtaattagaggaaacagaattagaatctctagggatttgagcccttaaacaattctacgataaactacaatttatacaatattttctgagtcatgtagttttgtgttggattgctttcggtctggtagaattcagctgggaaaccaactggtccagggcttttttggttggtaggtttttcattactgattccatttcagaagttgatattggtctattcacgttaacagtcttttcctgattcaatcttggaaaatcgtgtgcttacaggaaagtatccatttcctctagattttctaatttgtgtgcttagagttattcataatagtttctgaaggtcttttgtatttctgtgggaccagttatgatactgataaaaaaaaaaaccacctttttcatttctgattgtgctttcttggatcttctctttctttttctttgttaaactggctagtggcctatcgattttatttttttgaaaaaccaagtcttggttttattgatcttttgtatggatttttacatgtcaatttcattaagttcttctctaatttcagtggtttttcttctgctagttttggattttctcctccctagttcctttcccttagttgacctagtttcttcctttccaaagatagattgttaatttgagatttttttaacttcttgatgaagacatttagggctataaactttcctcttaacactgccttggctgcatccagagattttggtaagttgtgtccctattttcattaatttcaaacgatttttttgatttctgcctcaattttgatgttgacccaggagttatgctagagtaagttagttaatttcatgtatttgtatagtttgaggcaatcttgatattgatttctactattattgtactgtgattcaagaatgtgctttggtatgacttcaatcattttgaatttattgagactttttatgatcaagcatgtggttgatcttagaatacattctgtgtgcagacaagaaaaatgtatattttttggttgttgggtgtagtgtcctgtagctgtctgagatccagttggtcaagtgtcaagtttaaatccagagtttcattgttaactttctgccctgatgatctaacgctgtcagtaggatgttcaagcctcccactagtattttgtgtttgtctaaggtttttcgttggccaagaagaacttattttatgaatctgggtgctccaatgttgggtgcatatatatttagaacagttagggcttcttgttggattgtaccctttatcattatgtaatgccttttattgtccttcttgattttttatttaaagtctgttttatctgatataagtatagtgactcctgctcttttttcctctcagtttgcatggtagaattttctccattcttttactttgagcctgtgggtgttattatatgtgacatggatttcttgaagcaaactgacatttggggcttgtctttttatcaggctttccactctgtgacttttaagtgggcattaagcccatttatattcaaggttactattgatgggaatgattttaattttgtcattgtgttgttaactggctgttatgtagacttaattacgcagttgctttatagttcttgtgggctatggtctgaagtgtcttttgtggtagcaggctctttcaattctatgtttagcactccctcaccaggtccccctcaccggggacctgaggatctgaggactccctcaccaggtccacttctggggatgtcttgtaagtctggtctagtttaaatatactccctcagaatttgcttttctgagaaggattttatttcatcttcatttaagaagcttggtttggcagcatatgaaattcttggttagaattttttttcttcaagatgctaaaaataggcccccaatctcttctggcttataaggtttctgccgaaaggtctgctattagcctgatgggttccctttgtaagttacattccccatctttcttgctgcctttaagatgttttcttttgtgttcacttcagtgaatctgatgaccacgtgccttggggatggatgtcttgtatagtatctggctagggtcctctatatttcttggatttgcaggtcaacctctctaatgagtttagggaaattttcatggactatgtcctcaaatatactttccaagttgcttattatttttctttctcaagaatgccaatgagtcatagatttggtttctttgcataattgcatatttctcagaggttttgttcatttttctttattttttctctttatttttgcctgactgagttgacttaattaactgtcttcaagccctgaggttcttttctctgcttggtctattctgctgttaatagttctgcttgtagtttgaaattctcgtagcgaatttttcagttcaagaagttcaattttgggtctttcttaaaacggcttcttagtctttcaactcttgaatcattttactgaattgctttgcatccttggattgagtttcaactttctcttggtcttgataagcttcctagccatccagattctgaattctatgtctgccatttcagacatttcagactgattaaccattgctgggaacctagtgggcctgtttggaggtgaggggacactggctttctgaattgccagagttcttattctgatttttttcccatctgagaaggctgggttcctttaactgtgatggtaatctagcatagtcagttggctttgtatccggaagttttcagagggctaaggctctgtaagggtctttgtggttgaattcttgcccttggtttatcagcagggagaagtggcagagtgacttttttgttgttgttgtagtttgggctgcgatctggtagatagtgcttgagagcaatggatggaagacgggctcttacttggcagcatggctcctttgtgtatccttggatttgcagctatgctcctttcctcagacaccgctggaggccaggaagcagccttagcattcagttacccgcacggagtttccagcttcctccctcttcagcctcagggtctgcatcttttctacatccacattcagcatcttctttacaaagatctgtctgcttgttaagaaactgcacaacttccaaaccatcagggtaggtcgtgtgtgtcgtctgagcatttgcataatagtaaacatcacacgtaagttcacagcccaaatttcctgcagctctgcaatgtttggggaagaagcagtgaactcatcaggttgaacgtggctgagaaatccaccttcagaactctctaagactgaggagcttccgtctaaaaagcaaataagttaaatttaaaaggatagtgtatatacattgtggaaatatcagtatcctaatgcgattgctaaattcaatttaagcaaacgtgtgaacacattctttcttgttcatgagattactatacacatgtcaggtcagttcaacaacaaatgatcctgtaaggaacattaattctttaatgaatacactcagtcggtatttctctttcgagtattctgatggatcaggagattcacggatggaaaggcactgtcttggccctgaagctgctcacagtcccgcagcaggcaaacacagaagagaaaagccgaatccctgtgacactggcttacgggacctatgaagggccacgggccattgtgaaggagcaccacaggcttccaggagagccaggagtcaggggagcttccccaggatggcgtcactgtcagctgagatgatgcctggaggttgcggagatactagcaggtgtgtgtgagaggcaaggtcccccattctgcccggcaccagcaagtacactgaagtcttgtccgggggcctgaaggggaggggacagcaggaacaaggtagccaggctggagcagacctgatgggaagggcttccctgccccacagagaagtgcagaggggactgtgagggcacgcagagcctgaggtggtctgaagcagacagatggcaccagcctcacctctacgaagctccctgcagaggccatgaaacagcctgggggtgggcaggaagcccggggggcagactcaggaggaagacagtgtcagattcggccctgaagggccacgcagacctcggccaaggatgggaaggagtccaggtgccaggcagcccagggcgagtggtgcccacaggcttgggctgtgctgtgcataagggccacacctgaagctcggccacacctgaggctcggccaccacataggccccgtttctttaccaagataggttcctgcagaggtcgtgaagctgctgtggtcatttgctggcagcgacgtgaagatagaattctttcctgactcaaccaggggcactctcgtctcctccccgtgagacccgcaatgcaggaagcacccacagctgcatggacagaactggggcctgggaaagaggccaggaaggtgccagatgagagggcgctccatcagggtggcagcaatgccatgggctggcaaatggagaaaggggaacaaagcacccaagtgcatctagccccagccacacgccttctgctgggagtgtgctcagagggaagtgaccgctaggattcggaatctccagtcacggcccctggagaccggcatgtgggctgtgtgtggggtggagggctgggggtgttggcaagtctcacaggtgaggacccaacgagggaatcagacaaaaagtggccacaaattaggcagctccaggaaggacatgtccttgccatagtaagatgttctgctcacgcgtatccacgagaaagccccgcatttcacggggagcatagaaacaggagtccccaactctgctcaccagctcctccggctgctgccatctgctcctgcagcatggcggcctgggaagcctgcactggtgattttctgccactcaagttttgcagacttcgggaagatggatgcatagcctggggcaatgacagtcacaggcccgccttgtcacaaggtccctggagcgggcaatgccttgagcccaaaggctgggagcacaaagccatcttcagccatcctcgatttccagcaagaccccagggctcacccaacagcccgacactccatactacaaggtgggttaatttttttaaagactctgcagaaatataccaactacagagctcaggaaagcaactgatttataaaacccaatccaagttgtttgcttttatagcattagagacatgtctgaagaacttcaagtttttatctatagaaacataattagtttaataaattactaggtctattttgaataacaaattgagtacttttattagacctaagtggaactttatctgaatctgaattttccaaggggccagtgtagagtgacacaggtgtccgaggccacctttccatcttcagacacccccccgtctctctgcacagggagttggccttccagtaggtgttgctcttctgtcttgacgtctcctggaaagatttttatctctattttcctgtggtggtgttttccacgagctaattctttctatctttaaactcattggctttggaggagctgaattgttagatgacgatctttgtcccaggagagtggcactctgattcttgtggccagcgtatttgggtattgtctcttcatcagctgacagaggtgaaatttttccaaaagcaggttccaatgccagagtgtgcgattcttgccccgcgtgtggggacgctgcagatttcttcctggctttccaccgctgcagctgcagagctctcagcttttctcggagctccatgttctgctccctcaaagcatctatatgactccggagttttccatgaacatcagcccacagagacttctgtctcccaagctcttggtggagtctgatgatctgctgctgtaatggttgctgaatcttggcgataattttggttttttcattcttccccacgtagtctgaaagcttcttcgttcttctcagctccttggctgcccaccacagctgcgcctctgcctctttaatgacgttgagccctgcctgtgttcccgacaagtcttccttattttcaaactccatgcggatgggatcatacggtggcaaccccatggggtaaacaatcatcaccgcgcctcgaagctggtccaaggcatctttcaccatctccatggtaacacagacaccggcttccacttgtttcttagatattattgctttggcttcttctatagtcttctttaacacttgcttcatcttctcatttggagcttgcccattccttcgtccaatatcatcctttttaaacactgcacctccgctgggtacgcatttttcaccccattcatccttcaatttcaattcttcaatctgatcatcggtcagtccttgcatattaggagggagaaatatgccatgttcggctaattcttccatttctgagcagaggcgctgcaccttgagccgcccattatagacccgggccacctgcaccgtgagctcctccagctcggtactcccaggcgcctgcagcaggaactggctctcgtcgccccgcttcacgtgcagcagaaccatggcggtcccgccgaggtactgaggcgttgagaaggccccggctgcgtggcccgcgggtcctgccggccgagggtcgccggatcgccagcagctgcgacgcactaacagccgctcacagtccggaatcccacgct

SEQ ID NO: 11336 - RNA, 7213 nt, Homo sapiens
  source 1..7213: mol_type = other RNA
ctgaatagctgggactacaggtgcccgccaccacgcctggctaattttttattttttgtatttttagtagagacagggtttcactatgttagccaggatggtctcgatctcctgacctcgtgatctgcctgccttggcctcccaaagtgctgggattacaggtgtgagccactgcgcccggccttttccttgacattttcaaagaactatgcatgtaatattatagtgactgttcacccagccccttgccctaaagcctggtaacatgattaactcatgattcctggataaatgctatgttctcattcctccatttttatctatacgtaaggctcttggctttgaattttatttctatctctttgtttggttaagttcatcttggtaaaacattagctctccccgcatttgttctcagttctatgatgtagagttgataaactttcccagtaggacagacacatattttgcccaatgtgtgttctctgtaaatgcaggtgaggaaggaggggtaattagaggaaacagaattagaatctctagggatttgagcccttaaacaattctacgataaactacaatttatacaatattttctgagtcatgtagttttgtgttggattgctttcggtctggtagaattcagctgggaaaccaactggtccagggcttttttggttggtaggtttttcattactgattccatttcagaagttgatattggtctattcacgttaacagtcttttcctgattcaatcttggaaaatcgtgtgcttacaggaaagtatccatttcctctagattttctaatttgtgtgcttagagttattcataatagtttctgaaggtcttttgtatttctgtgggaccagttatgatactgataaaaaaaaaaaccacctttttcatttctgattgtgctttcttggatcttctctttctttttctttgttaaactggctagtggcctatcgattttatttttttgaaaaaccaagtcttggttttattgatcttttgtatggatttttacatgtcaatttcattaagttcttctctaatttcagtggtttttcttctgctagttttggattttctcctccctagttcctttcccttagttgacctagtttcttcctttccaaagatagattgttaatttgagatttttttaacttcttgatgaagacatttagggctataaactttcctcttaacactgccttggctgcatccagagattttggtaagttgtgtccctattttcattaatttcaaacgatttttttgatttctgcctcaattttgatgttgacccaggagttatgctagagtaagttagttaatttcatgtatttgtatagtttgaggcaatcttgatattgatttctactattattgtactgtgattcaagaatgtgctttggtatgacttcaatcattttgaatttattgagactttttatgatcaagcatgtggttgatcttagaatacattctgtgtgcagacaagaaaaatgtatattttttggttgttgggtgtagtgtcctgtagctgtctgagatccagttggtcaagtgtcaagtttaaatccagagtttcattgttaactttctgccctgatgatctaacgctgtcagtaggatgttcaagcctcccactagtattttgtgtttgtctaaggtttttcgttggccaagaagaacttattttatgaatctgggtgctccaatgttgggtgcatatatatttagaacagttagggcttcttgttggattgtaccctttatcattatgtaatgccttttattgtccttcttgattttttatttaaagtctgttttatctgatataagtatagtgactcctgctcttttttcctctcagtttgcatggtagaattttctccattcttttactttgagcctgtgggtgttattatatgtgacatggatttcttgaagcaaactgacatttggggcttgtctttttatcaggctttccactctgtgacttttaagtgggcattaagcccatttatattcaaggttactattgatgggaatgattttaattttgtcattgtgttgttaactggctgttatgtagacttaattacgcagttgctttatagttcttgtgggctatggtctgaagtgtcttttgtggtagcaggctctttcaattctatgtttagcactccctcaccaggtccccctcaccggggacctgaggatctgaggactccctcaccaggtccacttctggggatgtcttgtaagtctggtctagtttaaatatactccctcagaatttgcttttctgagaaggattttatttcatcttcatttaagaagcttggtttggcagcatatgaaattcttggttagaattttttttcttcaagatgctaaaaataggcccccaatctcttctggcttataaggtttctgccgaaaggtctgctattagcctgatgggttccctttgtaagttacattccccatctttcttgctgcctttaagatgttttcttttgtgttcacttcagtgaatctgatgaccacgtgccttggggatggatgtcttgtatagtatctggctagggtcctctatatttcttggatttgcaggtcaacctctctaatgagtttagggaaattttcatggactatgtcctcaaatatactttccaagttgcttattatttttctttctcaagaatgccaatgagtcatagatttggtttctttgcataattgcatatttctcagaggttttgttcatttttctttattttttctctttatttttgcctgactgagttgacttaattaactgtcttcaagccctgaggttcttttctctgcttggtctattctgctgttaatagttctgcttgtagtttgaaattctcgtagcgaatttttcagttcaagaagttcaattttgggtctttcttaaaacggcttcttagtctttcaactcttgaatcattttactgaattgctttgcatccttggattgagtttcaactttctcttggtcttgataagcttcctagccatccagattctgaattctatgtctgccatttcagacatttcagactgattaaccattgctgggaacctagtgggcctgtttggaggtgaggggacactggctttctgaattgccagagttcttattctgatttttttcccatctgagaaggctgggttcctttaactgtgatggtaatctagcatagtcagttggctttgtatccggaagttttcagagggctaaggctctgtaagggtctttgtggttgaattcttgcccttggtttatcagcagggagaagtggcagagtgacttttttgttgttgttgtagtttgggctgcgatctggtagatagtgcttgagagcaatggatggaagacgggctcttacttggcagcatggctcctttgtgtatccttggatttgcagctatgctcctttcctcagacaccgctggaggccaggaagcagccttagcattcagttacccgcacggagtttccagcttcctccctcttcagcctcagggtctgcatcttttctacatccacattcagcatcttctttacaaagatctgtctgcttgttaagaaactgcacaacttccaaaccatcagggtaggtcgtgtgtgtcgtctgagcatttgcataatagtaaacctgcagctctgcaatgtttggggaagaagcagtgaactcatcaggttgaacgtggctgagaaatccaccttcagaactctctaagactgaggagcttccgtctaaaaagcaaataagttaaatttaaaaggatagtgtatatacattgtggaaatatcagtatcctaatgcgattgctaaattcaatttaagcaaacgtgtgaacacattctttcttgttcatgagattactatacacatgtcaggtcagttcaacaacaaatgatcctgtaaggaacattaattctttaatgaatacactcagtcggtatttctctttcgagtattctgatggatcaggagattcacggatggaaaggcactgtcttggccctgaagctgctcacagtcccgcagcaggcaaacacagaagagaaaagccgaatccctgtgacactggcttacgggacctatgaagggccacgggccattgtgaaggagcaccacaggcttccaggagagccaggagtcaggggagcttccccaggatggcgtcactgtcagctgagatgatgcctggaggttgcggagatactagcaggtgtgtgtgagaggcaaggtcccccattctgcccggcaccagcaagtacactgaagtcttgtccgggggcctgaaggggaggggacagcaggaacaaggtagccaggctggagcagacctgatgggaagggcttccctgccccacagagaagtgcagaggggactgtgagggcacgcagagcctgaggtggtctgaagcagacagatggcaccagcctcacctctacgaagctccctgcagaggccatgaaacagcctgggggtgggcaggaagcccggggggcagactcaggaggaagacagtgtcagattcggccctgaagggccacgcagacctcggccaaggatgggaaggagtccaggtgccaggcagcccagggcgagtggtgcccacaggcttgggctgtgctgtgcataagggccacacctgaagctcggccacacctgaggctcggccaccacataggccccgtttctttaccaagataggttcctgcagaggtcgtgaagctgctgtggtcatttgctggcagcgacgtgaagatagaattctttcctgactcaaccaggggcactctcgtctcctccccgtgagacccgcaatgcaggaagcacccacagctgcatggacagaactggggcctgggaaagaggccaggaaggtgccagatgagagggcgctccatcagggtggcagcaatgccatgggctggcaaatggagaaaggggaacaaagcacccaagtgcatctagccccagccacacgccttctgctgggagtgtgctcagagggaagtgaccgctaggattcggaatctccagtcacggcccctggagaccggcatgtgggctgtgtgtggggtggagggctgggggtgttggcaagtctcacaggtgaggacccaacgagggaatcagacaaaaagtggccacaaattaggcagctccaggaaggacatgtccttgccatagtaagatgttctgctcacgcgtatccacgagaaagccccgcatttcacggggagcatagaaacaggagtccccaactctgctcaccagctcctccggctgctgccatctgctcctgcagcatggcggcctgggaagcctgcactggtgattttctgccactcaagttttgcagacttcgggaagatggatgcatagcctggggcaatgacagtcacaggcccgccttgtcacaaggtccctggagcgggcaatgccttgagcccaaaggctgggagcacaaagccatcttcagccatcctcgatttccagcaagaccccagggctcacccaacagcccgacactccatactacaaggtgggttaatttttttaaagactctgcagaaatataccaactacagagctcaggaaagcaactgatttataaaacccaatccaagttgtttgcttttatagcattagagacatgtctgaagaacttcaagtttttatctatagaaacataattagtttaataaattactaggtctattttgaataacaaattgagtacttttattagacctaagtggaactttatctgaatctgaattttccaaggggccagtgtagagtgacacaggtgtccgaggccacctttccatcttcagacacccccccgtctctctgcacagggagttggccttccagtaggtgttgctcttctgtcttgacgtctcctggaaagatttttatctctattttcctgtggtggtgttttccacgagctaattctttctatctttaaactcattggctttggaggagctgaattgttagatgacgatctttgtcccaggagagtggcactctgattcttgtggccagcgtatttgggtattgtctcttcatcagctgacagaggtgaaatttttccaaaagcaggttccaatgccagagtgtgcgattcttgccccgcgtgtggggacgctgcagatttcttcctggctttccaccgctgcagctgcagagctctcagcttttctcggagctccatgttctgctccctcaaagcatctatatgactccggagttttccatgaacatcagcccacagagacttctgtctcccaagctcttggtggagtctgatgatctgctgctgtaatggttgctgaatcttggcgataattttggttttttcattcttccccacgtagtctgaaagcttcttcgttcttctcagctccttggctgcccaccacagctgcgcctctgcctctttaatgacgttgagccctgcctgtgttcccgacaagtcttccttattttcaaactccatgcggatgggatcatacggtggcaaccccatggggtaaacaatcatcaccgcgcctcgaagctggtccaaggcatctttcaccatctccatggtaacacagacaccggcttccacttgtttcttagatattattgctttggcttcttctatagtcttctttaacacttgcttcatcttctcatttggagcttgcccattccttcgtccaatatcatcctttttaaacactgcacctccgctgggtacgcatttttcaccccattcatccttcaatttcaattcttcaatctgatcatcggtcagtccttgcatattaggagggagaaatatgccatgttcggctaattcttccatttctgagcagaggcgctgcaccttgagccgcccattatagacccgggccacctgcaccgtgagctcctccagctcggtactcccaggcgcctgcagcaggaactggctctcgtcgccccgcttcacgtgcagcagaaccatggcggtcccgccgaggtactgaggcgttgagaaggccccggctgcgtggcccgcgggtcctgccggccgagggtcgccggatcgccagcagctgcgacgcactaacagccgctcacagtccggaatcccacgct

SEQ ID NO: 11337 - RNA, 6616 nt, Homo sapiens
  source 1..6616: mol_type = other RNA
ctgaatagctgggactacaggtgcccgccaccacgcctggctaattttttgtatttttagtagagacggggtttcaccatgttagccaggatggtcttgatttcctgacctcatgatctgcccacctcggcctcccaaagtgctgggattacaggtatgagccactgcgcctggcccatttagtatgatctttacaataattctgtgaagaaagaattcttaccctctttttttcccatttatttatttatattattttttgagacggagtctcgctctgtcacccaggctggagtgcaatggtgcaatcttagctcactgcaaactccacctctcaggttccaattctcctgcctcagcctccagagtagctggaattacaggcacgccaccatgcccagctatttttttgtatttttagtagatacggggttttgtcatgttggccagactggtcttgaactcctgacctcaggtgatccatttgccttggcctcccaaagtgccgggattacacgcatgagccacatctggctttttttcatttattgataaatgaaattttgcatattatggggtgcatatgaatgtgttttatatacacagaatgtgtaattatcaagccagggtatttgaggtattcaccaccttgagaatttataattttatgtgttgggaacatttcaagttctctcttctagcaactttgaaatacacaatatattgttgctaactgtagccaccctagtctgctaccaaacattagaaggtatttcttccctaagtttgtacccattcaccaacctatcaagaagttttactattttacaggtgaggaaactcaggttcagagaggctaggtcatttgtccaaggtcattgctgttacacagcagaggcaggatttaaaccctggcttgctcaactccggagttggtgggtttttttttctttagaaatagcgtctctgtctgtaaggctgtgagggtgtagtgcagtggcacaatcacagttcactgcagcctagaattccttcgcttaggcgatgctcccgacccagcctcctgagtagctgggagtacaggtgcatgacacacctggctaattaaaaaaaagttttttagagatagggtctctgtatgttgcccaggctgatctcaaactcctgtcctcaagtaatcctcctgcctttgcctcccaaagtgctgggatcacaggtatgagccaccacatccaacccagagtttgtgctcttaaccagggatgacatgttgcaacttcactcctcacagtgtggcccacagacgagcatcatcagcatcacccgggagcttgttaaactgcagcatcaggccacatccagggcctgagtcagaatctgtattttgacaagatcccaagtgattcgtgtgcatactagtttgagaagctttggggaccacagtttcactaatggttttttttttttaatttcttttgagacggagtttcattcttgttgcccagggtagagtgcaatggcgcagtcttggctcactgcaacctccacctcccgggttgtagagattctcctgcctcagcctcctaagtagctgggattacaggcgaccgccaccacgcccagctaatttttttttttttttttgtatttttagtagagacggggtttcaccatgttggccaggctggtctcgaactcctgaccttaggtgatccacccacctcggcctcccaaaatgctggaattacaggtgtgagccactgtgcctggctttgttggttttaacagttctttcccatgcaggctgcagctgaacagccaagtcccctccttgggtcacatatttttctgaaaatgttataaaaaaattgagtccactggcctgggctaattacctagcagaacatccccatggtttggtgattctgaatatcgctgccaaacaagcacttgtagaggctcaaacaaggccataaaacatggcaatgggggcgcgctcccactctgggaaatgaaaatctgacgatactttgaattacagtggatcaagattaattccaggctctacttagaggaagctttcaggcccagtggtttagacataaaagcagtttgccctaatgcggcaggtgaaagctgtgacaactctattgcttggtgccaattacatttatggacttgtacccaggagtgctaggaaattgtcaccattagtgctgacgtactgccagttgttggctctgtctagtggggttctgatttgaagactcattattaatattccctgtagtgatctgcaatgctgctccattatggcaagtctgtcaggaacggagtttgtgtaggaattttagaaaacagcaataggttgagggctatgtggtaggccccagagcttctcaaactactgtgcacacaaatcacccagggtctcgttgagatgcagattcggaatcacgtcctgagctgaggcttgatacttttcttcttttttggagacaggatctctctctgttgcccaggccagagtgcaatggtgcagtcatggctcactgcagcctcaaattcttaggctcaagcaatcctctcaccttgccttctgagtagttgggactacaggcgttagccactacgcctggcttttttttttttttgagatggagttttgctcttgttgcccaggctagagtgcaatggcatggtcttggctcactgcaacctctgcctcctgggttcaagtgattctcctgcctcagcctcccaagtagctgggattacaggcatgagccaccacacccggctaattttgtatttttagtagaggcagggtttcaccatgttggccaggctggtcttgaactcctgactttgggtgatccacccgcctcggcctcccaaagtgctgggatgacaggcatgagccaccatgcccggcacctcgcctggctttttaatttttgagatgtctggctctgttgcccaggctggagggcagtgttgcgatcttggctcactgcaaccttcgcctcccaggttcaagcgattctcctgcctcggcctcccaagtagctgggactgcaggcgcaaaccaccatgccagactaattggctgtttaatttttaatagagatggggtcttgctttgttgtccaggctggttgaactcctggccttaattgatcctcctgccttggcctcccaaagtatcgggattgcaggagtgagccaacatgctcagcctgatgttgcatttctaaccagcatccacgtgatgccacagatgctgctgctgctccagcgggaatgtgggaaaagcacaggctcaggagtcagatggacatgggtggacatgggctctaaacctgactctgcccttggttgctgtgtgatgttgggcaagttgctgaacctctctgaattttggatttctcatgtgcaaaatagggatcacttctgccttttaggttctttgaagatttataataacgtacatgcataggttttcttcttgctcccagaggggcagggtgaggtcactctcctgcatgctctcactacaggttcagctgagaccgtttttcttctctaaagtacttggctttcttcttccaagtcaggatttctccgcctcggcgctactcacattttgggctggatcattttgtgttgtgggggatgctccgtgattaccgcattatagaacgttcagcagcatctctggcctcacccactggatactggtggcacccgtctcccctacttgtgaccaccgaaaatgtctccaggcactgccaaatgttcctggaggcaaaatcactcacaaataggaaataatgacctaattagtaacttacattagcaattcattcaacaatatgtgttgagcatctactgtttgccagaccatacagcagggatgtagtgatatttaagacaaacaaggtccctgacctcatggagactttttcctttttggacctcagtcttctccgctgtaatgtgggtatcacaaggctgcggacctcctaaatttgttgggaagatgaagttagacttgcaagtgcctggcccctggcatgagggattagccaatgccaggggtatgatgggcctagggatggaacctgggagcttggggagaagcgagtgtgggcagggacagtgcatggagaagccaggaaacctgagctgcaagggaggcggaaaggggccatgaaaggccctggtgcaaagtgtgcggcagcagcaaggcaggggaaaggggctgcagggagggccaagggtagcaggaagatgggaccaaaactggagagaaggagagagacagtgggacatagaggatgacaggaaggggtggagatgggaggagagaggcacagatggagaagataaaaaaccagacagacagacatgtacacacgtgataagacagagagaccaaggggcggagggaaaatgagtccaggcggaagggaacacctctgaggaagatcactgcacaaaccctggtcagctgcacatgaccccaaagagtggctcttaggtttattccaaacgtacctgatttgggtgataaagagttaaaattaaatacaaaggccaatgccagtccattcctggcgccagctcctgcctcttccttctcatggggccctcaccagagtgatggggtggagcatacccaaccctgggaggaaatgaggcttttgtgccgagcggcaatatgatggcaatactggcagtggtagtcaacccatctgtaaacagctgacagagggcagtacaagaatccacctcacagccagggccgcaaccgcaagtaaagcacacagctgaaatgactgacgtgggtggaactgagctgagaaggaacgtggctcggcttgaccctggagcacacatcacaaccatgagaaacaggcaactaaagtgacctccagcccacagcaacaaccttctctggctacaactgggaggcagggacagaccccagaaaaccatcttgggtcatctaaggtacgtgtaaccatatttttaaaatgacaaaatctcaagcatgttgctttggtgagcttctgattttactagaaatacactctaagaacagtcgagacgccgcgccttgtggaggcgatgggtcatgttactggttctgcgatgatcttccagagctccagttgctggaggcgctcgtaaaccaggagctgtgggaaggaggcctccacgggctccaccacgaagcgcagcttgccatctgcgagctgctccagcgcgtgcaggcaggagcggaagtgatcgtaggcttcacatgtgacgtccaagtgtctcaatgtgaagttgagcctgcaaaccagccagtcggacgcacaaactcttctccaccgacagtatggctgtgcaggcatttttcaatctgtgggcgagtcgggagagcgttttaaacacagcatcagtcaagtcgtcgtcgtaaaacacttcggctgcaaacaggatggtggtgtgatcgtacaagtcagaaatttcctcttgtgaccaactgaaggggaccttgggatctgtgcagaggtcgtccttcagccagtccagttctttgaccctaactataccacctccagtggcagccaggtggctgttgagggcaatgtttcgctggcacatggacaagagatctgcaccgacatctgtacaataaacggtccgtgccatggtggctgcgatgatgctagcgagccccgtgccggccccgagctccagcgctgtacatcctcggaagaggtcctgtcggaacaggatgtagtctgccaggagcagggcgccccgccacacctattctgatgatatcgtgcgggctgccttgtgcttcctctcccaggacgtcgtcttcttcctgtgctagaatcatgggatgtaccttgtctctcagaggccctgctgggttggaatcagaggcggctcgtggtcttctcaccacgtccaaatccccatcctcatccagctgagcttcagccacttcctggccagtggtgtcagtcccggcctggagggagaaaccctcattaccatggccacttcctggaggggaccctgtgctgcctgtctcagcagaaggaggctcctttgtgtgaacatctctgtgactgccacccttggctcctgaatctgtccaagagtcttggctccatagaagcttgaattgggacaggaaaactggctgccccacgctgttcagccgtaccatgagatgtctatggttcggggtatagaggtggacatctgacagcacagtgtcgctcctaaaggtgacctcgtccatggctgccgcaggagccagctgtaccatggcccaggctccaccttagtcctaggacaggagtccctcagaggtgagaatgggtcctcagcatggcaggtcccagaggagatactgcagacaggtccaagctggtagcgagtagctttgcatcgccctgggagaagatctcagagacttggccagggaagagaatccagccgccgcggggcccagcctgggatcccacccgactcccgtctctgtgggacttaggcggccgccataacaggcggtctgcgcaggcgcggccccgcccccgcgtgc

SEQ ID NO: 11338 - RNA, 6657 nt, Homo sapiens
  source 1..6657: mol_type = other RNA
ctgaatagctgggactacaggtgcccgccaccacgcctggctaattttttgtatttttagtagagacggggtttcaccatgttagccaggatggtcttgatttcctgacctcatgatctgcccacctcggcctcccaaagtgctgggattacaggtatgagccactgcgcctggcccatttagtatgatctttacaataattctgtgaagaaagaattcttaccctctttttttcccatttatttatttatattattttttgagacggagtctcgctctgtcacccaggctggagtgcaatggtgcaatcttagctcactgcaaactccacctctcaggttccaattctcctgcctcagcctccagagtagctggaattacaggcacgccaccatgcccagctatttttttgtatttttagtagatacggggttttgtcatgttggccagactggtcttgaactcctgacctcaggtgatccatttgccttggcctcccaaagtgccgggattacacgcatgagccacatctggctttttttcatttattgataaatgaaattttgcatattatggggtgcatatgaatgtgttttatatacacagaatgtgtaattatcaagccagggtatttgaggtattcaccaccttgagaatttataattttatgtgttgggaacatttcaagttctctcttctagcaactttgaaatacacaatatattgttgctaactgtagccaccctagtctgctaccaaacattagaaggtatttcttccctaagtttgtacccattcaccaacctatcaagaagttttactattttacaggtgaggaaactcaggttcagagaggctaggtcatttgtccaaggtcattgctgttacacagcagaggcaggatttaaaccctggcttgctcaactccggagttggtgggtttttttttctttagaaatagcgtctctgtctgtaaggctgtgagggtgtagtgcagtggcacaatcacagttcactgcagcctagaattccttcgcttaggcgatgctcccgacccagcctcctgagtagctgggagtacaggtgcatgacacacctggctaattaaaaaaaagttttttagagatagggtctctgtatgttgcccaggctgatctcaaactcctgtcctcaagtaatcctcctgcctttgcctcccaaagtgctgggatcacaggtatgagccaccacatccaacccagagtttgtgctcttaaccagggatgacatgttgcaacttcactcctcacagtgtggcccacagacgagcatcatcagcatcacccgggagcttgttaaactgcagcatcaggccacatccagggcctgagtcagaatctgtattttgacaagatcccaagtgattcgtgtgcatactagtttgagaagctttggggaccacagtttcactaatggttttttttttttaatttcttttgagacggagtttcattcttgttgcccagggtagagtgcaatggcgcagtcttggctcactgcaacctccacctcccgggttgtagagattctcctgcctcagcctcctaagtagctgggattacaggcgaccgccaccacgcccagctaatttttttttttttttttgtatttttagtagagacggggtttcaccatgttggccaggctggtctcgaactcctgaccttaggtgatccacccacctcggcctcccaaaatgctggaattacaggtgtgagccactgtgcctggctttgttggttttaacagttctttcccatgcaggctgcagctgaacagccaagtcccctccttgggtcacatatttttctgaaaatgttataaaaaaattgagtccactggcctgggctaattacctagcagaacatccccatggtttggtgattctgaatatcgctgccaaacaagcacttgtagaggctcaaacaaggccataaaacatggcaatgggggcgcgctcccactctgggaaatgaaaatctgacgatactttgaattacagtggatcaagattaattccaggctctacttagaggaagctttcaggcccagtggtttagacataaaagcagtttgccctaatgcggcaggtgaaagctgtgacaactctattgcttggtgccaattacatttatggacttgtacccaggagtgctaggaaattgtcaccattagtgctgacgtactgccagttgttggctctgtctagtggggttctgatttgaagactcattattaatattccctgtagtgatctgcaatgctgctccattatggcaagtctgtcaggaacggagtttgtgtaggaattttagaaaacagcaataggttgagggctatgtggtaggccccagagcttctcaaactactgtgcacacaaatcacccagggtctcgttgagatgcagattcggaatcacgtcctgagctgaggcttgatacttttcttcttttttggagacaggatctctctctgttgcccaggccagagtgcaatggtgcagtcatggctcactgcagcctcaaattcttaggctcaagcaatcctctcaccttgccttctgagtagttgggactacaggcgttagccactacgcctggcttttttttttttttgagatggagttttgctcttgttgcccaggctagagtgcaatggcatggtcttggctcactgcaacctctgcctcctgggttcaagtgattctcctgcctcagcctcccaagtagctgggattacaggcatgagccaccacacccggctaattttgtatttttagtagaggcagggtttcaccatgttggccaggctggtcttgaactcctgactttgggtgatccacccgcctcggcctcccaaagtgctgggatgacaggcatgagccaccatgcccggcacctcgcctggctttttaatttttgagatgtctggctctgttgcccaggctggagggcagtgttgcgatcttggctcactgcaaccttcgcctcccaggttcaagcgattctcctgcctcggcctcccaagtagctgggactgcaggcgcaaaccaccatgccagactaattggctgtttaatttttaatagagatggggtcttgctttgttgtccaggctggttgaactcctggccttaattgatcctcctgccttggcctcccaaagtatcgggattgcaggagtgagccaacatgctcagcctgatgttgcatttctaaccagcatccacgtgatgccacagatgctgctgctgctccagcgggaatgtgggaaaagcacaggctcaggagtcagatggacatgggtggacatgggctctaaacctgactctgcccttggttgctgtgtgatgttgggcaagttgctgaacctctctgaattttggatttctcatgtgcaaaatagggatcacttctgccttttaggttctttgaagatttataataacgtacatgcataggttttcttcttgctcccagaggggcagggtgaggtcactctcctgcatgctctcactacaggttcagctgagaccgtttttcttctctaaagtacttggctttcttcttccaagtcaggatttctccgcctcggcgctactcacattttgggctggatcattttgtgttgtgggggatgctccgtgattaccgcattatagaacgttcagcagcatctctggcctcacccactggatactggtggcacccgtctcccctacttgtgaccaccgaaaatgtctccaggcactgccaaatgttcctggaggcaaaatcactcacaaataggaaataatgacctaattagtaacttacattagcaattcattcaacaatatgtgttgagcatctactgtttgccagaccatacagcagggatgtagtgatatttaagacaaacaaggtccctgacctcatggagactttttcctttttggacctcagtcttctccgctgtaatgtgggtatcacaaggctgcggacctcctaaatttgttgggaagatgaagttagacttgcaagtgcctggcccctggcatgagggattagccaatgccaggggtatgatgggcctagggatggaacctgggagcttggggagaagcgagtgtgggcagggacagtgcatggagaagccaggaaacctgagctgcaagggaggcggaaaggggccatgaaaggccctggtgcaaagtgtgcggcagcagcaaggcaggggaaaggggctgcagggagggccaagggtagcaggaagatgggaccaaaactggagagaaggagagagacagtgggacatagaggatgacaggaaggggtggagatgggaggagagaggcacagatggagaagataaaaaaccagacagacagacatgtacacacgtgataagacagagagaccaaggggcggagggaaaatgagtccaggcggaagggaacacctctgaggaagatcactgcacaaaccctggtcagctgcacatgaccccaaagagtggctcttaggtttattccaaacgtacctgatttgggtgataaagagttaaaattaaatacaaaggccaatgccagtccattcctggcgccagctcctgcctcttccttctcatggggccctcaccagagtgatggggtggagcatacccaaccctgggaggaaatgaggcttttgtgccgagcggcaatatgatggcaatactggcagtggtagtcaacccatctgtaaacagctgacagagggcagtacaagaatccacctcacagccagggccgcaaccgcaagtaaagcacacagctgaaatgactgacgtgggtggaactgagctgagaaggaacgtggctcggcttgaccctggagcacacatcacaaccatgagaaacaggcaactaaagtgacctccagcccacagcaacaaccttctctggctacaactgggaggcagggacagaccccagaaaaccatcttgggtcatctaaggtacgtgtaaccatatttttaaaatgacaaaatctcaagcatgttgctttggtgagcttctgattttactagaaatacactctaagaacagtcgagacgccgcgccttgtggaggcgatgggtcatgttactggttctgcgatgatcttccagagctccagttgctggaggcgctcgtaaaccaggagctgtgggaaggaggcctccacgggctccaccacgaagcgcagcttgccatctgcgagctgctccagcgcgtgcaggcaggagcggaagtgatcgtaggcttcacatgtgacgtccaagtgtctcaatgtgaagttgagcctgcaaaccagccagtcggacgcacaaactcttctccaccgacagtatggctgtgcaggcatttttcaatctgtgggcgagtcgggagagcgttttaaacacagcatcagtcaagtcgtcgtcgtaaaacacttcggctgcaaacaggatggtggtgtgatcgtacaagtcagaaatttcctcttgtgaccaactgaaggggaccttgggatctgtgcagaggtcgtccttcagccagtccagttctttgaccctaactataccacctccagtggcagccaggtggctgttgagggcaatgtttcgctggcacatggacaagagatctgcaccgacatctgtacaataaacggtccgtgccatggtggctgcgatgatgctagcgagccccgtgccggccccgagctccagcgctgtacatcctcggaagaggtcctgtcggaacaggatgtagtctgccaggagcagggcgccccgccacacctgcttgccaacatcctccaggggcgtggccatggtgtgctctattctgatgatatcgtgcgggctgccttgtgcttcctctcccaggacgtcgtcttcttcctgtgctagaatcatgggatgtaccttgtctctcagaggccctgctgggttggaatcagaggcggctcgtggtcttctcaccacgtccaaatccccatcctcatccagctgagcttcagccacttcctggccagtggtgtcagtcccggcctggagggagaaaccctcattaccatggccacttcctggaggggaccctgtgctgcctgtctcagcagaaggaggctcctttgtgtgaacatctctgtgactgccacccttggctcctgaatctgtccaagagtcttggctccatagaagcttgaattgggacaggaaaactggctgccccacgctgttcagccgtaccatgagatgtctatggttcggggtatagaggtggacatctgacagcacagtgtcgctcctaaaggtgacctcgtccatggctgccgcaggagccagctgtaccatggcccaggctccaccttagtcctaggacaggagtccctcagaggtgagaatgggtcctcagcatggcaggtcccagaggagatactgcagacaggtccaagctggtagcgagtagctttgcatcgccctgggagaagatctcagagacttggccagggaagagaatccagccgccgcggggcccagcctgggatcccacccgactcccgtctctgtgggacttaggcggccgccataacaggcggtctgcgcaggcgcggccccgcccccgcgtgc

SEQ ID NO: 11339 - RNA, 6419 nt, Homo sapiens
  source 1..6419: mol_type = other RNA
ctgaatagctgggactacaggtgcccgccaccacgcctggctaattttttgtatttttagtagagacggggtttcaccatgttagccaggatggtcttgatttcctgacctcatgatctgcccacctcggcctcccaaagtgctgggattacaggtatgagccactgcgcctggcccatttagtatgatctttacaataattctgtgaagaaagaattcttaccctctttttttcccatttatttatttatattattttttgagacggagtctcgctctgtcacccaggctggagtgcaatggtgcaatcttagctcactgcaaactccacctctcaggttccaattctcctgcctcagcctccagagtagctggaattacaggcacgccaccatgcccagctatttttttgtatttttagtagatacggggttttgtcatgttggccagactggtcttgaactcctgacctcaggtgatccatttgccttggcctcccaaagtgccgggattacacgcatgagccacatctggctttttttcatttattgataaatgaaattttgcatattatggggtgcatatgaatgtgttttatatacacagaatgtgtaattatcaagccagggtatttgaggtattcaccaccttgagaatttataattttatgtgttgggaacatttcaagttctctcttctagcaactttgaaatacacaatatattgttgctaactgtagccaccctagtctgctaccaaacattagaaggtatttcttccctaagtttgtacccattcaccaacctatcaagaagttttactattttacaggtgaggaaactcaggttcagagaggctaggtcatttgtccaaggtcattgctgttacacagcagaggcaggatttaaaccctggcttgctcaactccggagttggtgggtttttttttctttagaaatagcgtctctgtctgtaaggctgtgagggtgtagtgcagtggcacaatcacagttcactgcagcctagaattccttcgcttaggcgatgctcccgacccagcctcctgagtagctgggagtacaggtgcatgacacacctggctaattaaaaaaaagttttttagagatagggtctctgtatgttgcccaggctgatctcaaactcctgtcctcaagtaatcctcctgcctttgcctcccaaagtgctgggatcacaggtatgagccaccacatccaacccagagtttgtgctcttaaccagggatgacatgttgcaacttcactcctcacagtgtggcccacagacgagcatcatcagcatcacccgggagcttgttaaactgcagcatcaggccacatccagggcctgagtcagaatctgtattttgacaagatcccaagtgattcgtgtgcatactagtttgagaagctttggggaccacagtttcactaatggttttttttttttaatttcttttgagacggagtttcattcttgttgcccagggtagagtgcaatggcgcagtcttggctcactgcaacctccacctcccgggttgtagagattctcctgcctcagcctcctaagtagctgggattacaggcgaccgccaccacgcccagctaatttttttttttttttttgtatttttagtagagacggggtttcaccatgttggccaggctggtctcgaactcctgaccttaggtgatccacccacctcggcctcccaaaatgctggaattacaggtgtgagccactgtgcctggctttgttggttttaacagttctttcccatgcaggctgcagctgaacagccaagtcccctccttgggtcacatatttttctgaaaatgttataaaaaaattgagtccactggcctgggctaattacctagcagaacatccccatggtttggtgattctgaatatcgctgccaaacaagcacttgtagaggctcaaacaaggccataaaacatggcaatgggggcgcgctcccactctgggaaatgaaaatctgacgatactttgaattacagtggatcaagattaattccaggctctacttagaggaagctttcaggcccagtggtttagacataaaagcagtttgccctaatgcggcaggtgaaagctgtgacaactctattgcttggtgccaattacatttatggacttgtacccaggagtgctaggaaattgtcaccattagtgctgacgtactgccagttgttggctctgtctagtggggttctgatttgaagactcattattaatattccctgtagtgatctgcaatgctgctccattatggcaagtctgtcaggaacggagtttgtgtaggaattttagaaaacagcaataggttgagggctatgtggtaggccccagagcttctcaaactactgtgcacacaaatcacccagggtctcgttgagatgcagattcggaatcacgtcctgagctgaggcttgatacttttcttcttttttggagacaggatctctctctgttgcccaggccagagtgcaatggtgcagtcatggctcactgcagcctcaaattcttaggctcaagcaatcctctcaccttgccttctgagtagttgggactacaggcgttagccactacgcctggcttttttttttttttgagatggagttttgctcttgttgcccaggctagagtgcaatggcatggtcttggctcactgcaacctctgcctcctgggttcaagtgattctcctgcctcagcctcccaagtagctgggattacaggcatgagccaccacacccggctaattttgtatttttagtagaggcagggtttcaccatgttggccaggctggtcttgaactcctgactttgggtgatccacccgcctcggcctcccaaagtgctgggatgacaggcatgagccaccatgcccggcacctcgcctggctttttaatttttgagatgtctggctctgttgcccaggctggagggcagtgttgcgatcttggctcactgcaaccttcgcctcccaggttcaagcgattctcctgcctcggcctcccaagtagctgggactgcaggcgcaaaccaccatgccagactaattggctgtttaatttttaatagagatggggtcttgctttgttgtccaggctggttgaactcctggccttaattgatcctcctgccttggcctcccaaagtatcgggattgcaggagtgagccaacatgctcagcctgatgttgcatttctaaccagcatccacgtgatgccacagatgctgctgctgctccagcgggaatgtgggaaaagcacaggctcaggagtcagatggacatgggtggacatgggctctaaacctgactctgcccttggttgctgtgtgatgttgggcaagttgctgaacctctctgaattttggatttctcatgtgcaaaatagggatcacttctgccttttaggttctttgaagatttataataacgtacatgcataggttttcttcttgctcccagaggggcagggtgaggtcactctcctgcatgctctcactacaggttcagctgagaccgtttttcttctctaaagtacttggctttcttcttccaagtcaggatttctccgcctcggcgctactcacattttgggctggatcattttgtgttgtgggggatgctccgtgattaccgcattatagaacgttcagcagcatctctggcctcacccactggatactggtggcacccgtctcccctacttgtgaccaccgaaaatgtctccaggcactgccaaatgttcctggaggcaaaatcactcacaaataggaaataatgacctaattagtaacttacattagcaattcattcaacaatatgtgttgagcatctactgtttgccagaccatacagcagggatgtagtgatatttaagacaaacaaggtccctgacctcatggagactttttcctttttggacctcagtcttctccgctgtaatgtgggtatcacaaggctgcggacctcctaaatttgttgggaagatgaagttagacttgcaagtgcctggcccctggcatgagggattagccaatgccaggggtatgatgggcctagggatggaacctgggagcttggggagaagcgagtgtgggcagggacagtgcatggagaagccaggaaacctgagctgcaagggaggcggaaaggggccatgaaaggccctggtgcaaagtgtgcggcagcagcaaggcaggggaaaggggctgcagggagggccaagggtagcaggaagatgggaccaaaactggagagaaggagagagacagtgggacatagaggatgacaggaaggggtggagatgggaggagagaggcacagatggagaagataaaaaaccagacagacagacatgtacacacgtgataagacagagagaccaaggggcggagggaaaatgagtccaggcggaagggaacacctctgaggaagatcactgcacaaaccctggtcagctgcacatgaccccaaagagtggctcttaggtttattccaaacgtacctgatttgggtgataaagagttaaaattaaatacaaaggccaatgccagtccattcctggcgccagctcctgcctcttccttctcatggggccctcaccagagtgatggggtggagcatacccaaccctgggaggaaatgaggcttttgtgccgagcggcaatatgatggcaatactggcagtggtagtcaacccatctgtaaacagctgacagagggcagtacaagaatccacctcacagccagggccgcaaccgcaagtaaagcacacagctgaaatgactgacgtgggtggaactgagctgagaaggaacgtggctcggcttgaccctggagcacacatcacaaccatgagaaacaggcaactaaagtgacctccagcccacagcaacaaccttctctggctacaactgggaggcagggacagaccccagaaaaccatcttgggtcatctaaggtacgtgtaaccatatttttaaaatgacaaaatctcaagcatgttgctttggtgagcttctgattttactagaaatacactctaagaacagtcgagacgccgcgccttgtggaggcgatgggtcatgttactggttctgcgatgatcttccagagctcctcttctccaccgacagtatggctgtgcaggcatttttcaatctgtgggcgagtcgggagagcgttttaaacacagcatcagtcaagtcgtcgtcgtaaaacacttcggctgcaaacaggatggtggtgtgatcgtacaagtcagaaatttcctcttgtgaccaactgaaggggaccttgggatctgtgcagaggtcgtccttcagccagtccagttctttgaccctaactataccacctccagtggcagccaggtggctgttgagggcaatgtttcgctggcacatggacaagagatctgcaccgacatctgtacaataaacggtccgtgccatggtggctgcgatgatgctagcgagccccgtgccggccccgagctccagcgctgtacatcctcggaagaggtcctgtcggaacaggatgtagtctgccaggagcagggcgccccgccacacctattctgatgatatcgtgcgggctgccttgtgcttcctctcccaggacgtcgtcttcttcctgtgctagaatcatgggatgtaccttgtctctcagaggccctgctgggttggaatcagaggcggctcgtggtcttctcaccacgtccaaatccccatcctcatccagctgagcttcagccacttcctggccagtggtgtcagtcccggcctggagggagaaaccctcattaccatggccacttcctggaggggaccctgtgctgcctgtctcagcagaaggaggctcctttgtgtgaacatctctgtgactgccacccttggctcctgaatctgtccaagagtcttggctccatagaagcttgaattgggacaggaaaactggctgccccacgctgttcagccgtaccatgagatgtctatggttcggggtatagaggtggacatctgacagcacagtgtcgctcctaaaggtgacctcgtccatggctgccgcaggagccagctgtaccatggcccaggctccaccttagtcctaggacaggagtccctcagaggtgagaatgggtcctcagcatggcaggtcccagaggagatactgcagacaggtccaagctggtagcgagtagctttgcatcgccctgggagaagatctcagagacttggccagggaagagaatccagccgccgcggggcccagcctgggatcccacccgactcccgtctctgtgggacttaggcggccgccataacaggcggtctgcgcaggcgcggccccgcccccgcgtgc

SEQ ID NO: 11340 - RNA, 6460 nt, Homo sapiens
  source 1..6460: mol_type = other RNA
ctgaatagctgggactacaggtgcccgccaccacgcctggctaattttttgtatttttagtagagacggggtttcaccatgttagccaggatggtcttgatttcctgacctcatgatctgcccacctcggcctcccaaagtgctgggattacaggtatgagccactgcgcctggcccatttagtatgatctttacaataattctgtgaagaaagaattcttaccctctttttttcccatttatttatttatattattttttgagacggagtctcgctctgtcacccaggctggagtgcaatggtgcaatcttagctcactgcaaactccacctctcaggttccaattctcctgcctcagcctccagagtagctggaattacaggcacgccaccatgcccagctatttttttgtatttttagtagatacggggttttgtcatgttggccagactggtcttgaactcctgacctcaggtgatccatttgccttggcctcccaaagtgccgggattacacgcatgagccacatctggctttttttcatttattgataaatgaaattttgcatattatggggtgcatatgaatgtgttttatatacacagaatgtgtaattatcaagccagggtatttgaggtattcaccaccttgagaatttataattttatgtgttgggaacatttcaagttctctcttctagcaactttgaaatacacaatatattgttgctaactgtagccaccctagtctgctaccaaacattagaaggtatttcttccctaagtttgtacccattcaccaacctatcaagaagttttactattttacaggtgaggaaactcaggttcagagaggctaggtcatttgtccaaggtcattgctgttacacagcagaggcaggatttaaaccctggcttgctcaactccggagttggtgggtttttttttctttagaaatagcgtctctgtctgtaaggctgtgagggtgtagtgcagtggcacaatcacagttcactgcagcctagaattccttcgcttaggcgatgctcccgacccagcctcctgagtagctgggagtacaggtgcatgacacacctggctaattaaaaaaaagttttttagagatagggtctctgtatgttgcccaggctgatctcaaactcctgtcctcaagtaatcctcctgcctttgcctcccaaagtgctgggatcacaggtatgagccaccacatccaacccagagtttgtgctcttaaccagggatgacatgttgcaacttcactcctcacagtgtggcccacagacgagcatcatcagcatcacccgggagcttgttaaactgcagcatcaggccacatccagggcctgagtcagaatctgtattttgacaagatcccaagtgattcgtgtgcatactagtttgagaagctttggggaccacagtttcactaatggttttttttttttaatttcttttgagacggagtttcattcttgttgcccagggtagagtgcaatggcgcagtcttggctcactgcaacctccacctcccgggttgtagagattctcctgcctcagcctcctaagtagctgggattacaggcgaccgccaccacgcccagctaatttttttttttttttttgtatttttagtagagacggggtttcaccatgttggccaggctggtctcgaactcctgaccttaggtgatccacccacctcggcctcccaaaatgctggaattacaggtgtgagccactgtgcctggctttgttggttttaacagttctttcccatgcaggctgcagctgaacagccaagtcccctccttgggtcacatatttttctgaaaatgttataaaaaaattgagtccactggcctgggctaattacctagcagaacatccccatggtttggtgattctgaatatcgctgccaaacaagcacttgtagaggctcaaacaaggccataaaacatggcaatgggggcgcgctcccactctgggaaatgaaaatctgacgatactttgaattacagtggatcaagattaattccaggctctacttagaggaagctttcaggcccagtggtttagacataaaagcagtttgccctaatgcggcaggtgaaagctgtgacaactctattgcttggtgccaattacatttatggacttgtacccaggagtgctaggaaattgtcaccattagtgctgacgtactgccagttgttggctctgtctagtggggttctgatttgaagactcattattaatattccctgtagtgatctgcaatgctgctccattatggcaagtctgtcaggaacggagtttgtgtaggaattttagaaaacagcaataggttgagggctatgtggtaggccccagagcttctcaaactactgtgcacacaaatcacccagggtctcgttgagatgcagattcggaatcacgtcctgagctgaggcttgatacttttcttcttttttggagacaggatctctctctgttgcccaggccagagtgcaatggtgcagtcatggctcactgcagcctcaaattcttaggctcaagcaatcctctcaccttgccttctgagtagttgggactacaggcgttagccactacgcctggcttttttttttttttgagatggagttttgctcttgttgcccaggctagagtgcaatggcatggtcttggctcactgcaacctctgcctcctgggttcaagtgattctcctgcctcagcctcccaagtagctgggattacaggcatgagccaccacacccggctaattttgtatttttagtagaggcagggtttcaccatgttggccaggctggtcttgaactcctgactttgggtgatccacccgcctcggcctcccaaagtgctgggatgacaggcatgagccaccatgcccggcacctcgcctggctttttaatttttgagatgtctggctctgttgcccaggctggagggcagtgttgcgatcttggctcactgcaaccttcgcctcccaggttcaagcgattctcctgcctcggcctcccaagtagctgggactgcaggcgcaaaccaccatgccagactaattggctgtttaatttttaatagagatggggtcttgctttgttgtccaggctggttgaactcctggccttaattgatcctcctgccttggcctcccaaagtatcgggattgcaggagtgagccaacatgctcagcctgatgttgcatttctaaccagcatccacgtgatgccacagatgctgctgctgctccagcgggaatgtgggaaaagcacaggctcaggagtcagatggacatgggtggacatgggctctaaacctgactctgcccttggttgctgtgtgatgttgggcaagttgctgaacctctctgaattttggatttctcatgtgcaaaatagggatcacttctgccttttaggttctttgaagatttataataacgtacatgcataggttttcttcttgctcccagaggggcagggtgaggtcactctcctgcatgctctcactacaggttcagctgagaccgtttttcttctctaaagtacttggctttcttcttccaagtcaggatttctccgcctcggcgctactcacattttgggctggatcattttgtgttgtgggggatgctccgtgattaccgcattatagaacgttcagcagcatctctggcctcacccactggatactggtggcacccgtctcccctacttgtgaccaccgaaaatgtctccaggcactgccaaatgttcctggaggcaaaatcactcacaaataggaaataatgacctaattagtaacttacattagcaattcattcaacaatatgtgttgagcatctactgtttgccagaccatacagcagggatgtagtgatatttaagacaaacaaggtccctgacctcatggagactttttcctttttggacctcagtcttctccgctgtaatgtgggtatcacaaggctgcggacctcctaaatttgttgggaagatgaagttagacttgcaagtgcctggcccctggcatgagggattagccaatgccaggggtatgatgggcctagggatggaacctgggagcttggggagaagcgagtgtgggcagggacagtgcatggagaagccaggaaacctgagctgcaagggaggcggaaaggggccatgaaaggccctggtgcaaagtgtgcggcagcagcaaggcaggggaaaggggctgcagggagggccaagggtagcaggaagatgggaccaaaactggagagaaggagagagacagtgggacatagaggatgacaggaaggggtggagatgggaggagagaggcacagatggagaagataaaaaaccagacagacagacatgtacacacgtgataagacagagagaccaaggggcggagggaaaatgagtccaggcggaagggaacacctctgaggaagatcactgcacaaaccctggtcagctgcacatgaccccaaagagtggctcttaggtttattccaaacgtacctgatttgggtgataaagagttaaaattaaatacaaaggccaatgccagtccattcctggcgccagctcctgcctcttccttctcatggggccctcaccagagtgatggggtggagcatacccaaccctgggaggaaatgaggcttttgtgccgagcggcaatatgatggcaatactggcagtggtagtcaacccatctgtaaacagctgacagagggcagtacaagaatccacctcacagccagggccgcaaccgcaagtaaagcacacagctgaaatgactgacgtgggtggaactgagctgagaaggaacgtggctcggcttgaccctggagcacacatcacaaccatgagaaacaggcaactaaagtgacctccagcccacagcaacaaccttctctggctacaactgggaggcagggacagaccccagaaaaccatcttgggtcatctaaggtacgtgtaaccatatttttaaaatgacaaaatctcaagcatgttgctttggtgagcttctgattttactagaaatacactctaagaacagtcgagacgccgcgccttgtggaggcgatgggtcatgttactggttctgcgatgatcttccagagctcctcttctccaccgacagtatggctgtgcaggcatttttcaatctgtgggcgagtcgggagagcgttttaaacacagcatcagtcaagtcgtcgtcgtaaaacacttcggctgcaaacaggatggtggtgtgatcgtacaagtcagaaatttcctcttgtgaccaactgaaggggaccttgggatctgtgcagaggtcgtccttcagccagtccagttctttgaccctaactataccacctccagtggcagccaggtggctgttgagggcaatgtttcgctggcacatggacaagagatctgcaccgacatctgtacaataaacggtccgtgccatggtggctgcgatgatgctagcgagccccgtgccggccccgagctccagcgctgtacatcctcggaagaggtcctgtcggaacaggatgtagtctgccaggagcagggcgccccgccacacctgcttgccaacatcctccaggggcgtggccatggtgtgctctattctgatgatatcgtgcgggctgccttgtgcttcctctcccaggacgtcgtcttcttcctgtgctagaatcatgggatgtaccttgtctctcagaggccctgctgggttggaatcagaggcggctcgtggtcttctcaccacgtccaaatccccatcctcatccagctgagcttcagccacttcctggccagtggtgtcagtcccggcctggagggagaaaccctcattaccatggccacttcctggaggggaccctgtgctgcctgtctcagcagaaggaggctcctttgtgtgaacatctctgtgactgccacccttggctcctgaatctgtccaagagtcttggctccatagaagcttgaattgggacaggaaaactggctgccccacgctgttcagccgtaccatgagatgtctatggttcggggtatagaggtggacatctgacagcacagtgtcgctcctaaaggtgacctcgtccatggctgccgcaggagccagctgtaccatggcccaggctccaccttagtcctaggacaggagtccctcagaggtgagaatgggtcctcagcatggcaggtcccagaggagatactgcagacaggtccaagctggtagcgagtagctttgcatcgccctgggagaagatctcagagacttggccagggaagagaatccagccgccgcggggcccagcctgggatcccacccgactcccgtctctgtgggacttaggcggccgccataacaggcggtctgcgcaggcgcggccccgcccccgcgtgc

SEQ ID NO: 11341 - RNA, 6733 nt, Homo sapiens
  source 1..6733: mol_type = other RNA
ctgaatagctgggactacaggtgcccgccaccacgcctggctaattttttgtatttttagtagagacggggtttcaccatgttagccaggatggtcttgatttcctgacctcatgatctgcccacctcggcctcccaaagtgctgggattacaggtatgagccactgcgcctggcccatttagtatgatctttacaataattctgtgaagaaagaattcttaccctctttttttcccatttatttatttatattattttttgagacggagtctcgctctgtcacccaggctggagtgcaatggtgcaatcttagctcactgcaaactccacctctcaggttccaattctcctgcctcagcctccagagtagctggaattacaggcacgccaccatgcccagctatttttttgtatttttagtagatacggggttttgtcatgttggccagactggtcttgaactcctgacctcaggtgatccatttgccttggcctcccaaagtgccgggattacacgcatgagccacatctggctttttttcatttattgataaatgaaattttgcatattatggggtgcatatgaatgtgttttatatacacagaatgtgtaattatcaagccagggtatttgaggtattcaccaccttgagaatttataattttatgtgttgggaacatttcaagttctctcttctagcaactttgaaatacacaatatattgttgctaactgtagccaccctagtctgctaccaaacattagaaggtatttcttccctaagtttgtacccattcaccaacctatcaagaagttttactattttacaggtgaggaaactcaggttcagagaggctaggtcatttgtccaaggtcattgctgttacacagcagaggcaggatttaaaccctggcttgctcaactccggagttggtgggtttttttttctttagaaatagcgtctctgtctgtaaggctgtgagggtgtagtgcagtggcacaatcacagttcactgcagcctagaattccttcgcttaggcgatgctcccgacccagcctcctgagtagctgggagtacaggtgcatgacacacctggctaattaaaaaaaagttttttagagatagggtctctgtatgttgcccaggctgatctcaaactcctgtcctcaagtaatcctcctgcctttgcctcccaaagtgctgggatcacaggtatgagccaccacatccaacccagagtttgtgctcttaaccagggatgacatgttgcaacttcactcctcacagtgtggcccacagacgagcatcatcagcatcacccgggagcttgttaaactgcagcatcaggccacatccagggcctgagtcagaatctgtattttgacaagatcccaagtgattcgtgtgcatactagtttgagaagctttggggaccacagtttcactaatggttttttttttttaatttcttttgagacggagtttcattcttgttgcccagggtagagtgcaatggcgcagtcttggctcactgcaacctccacctcccgggttgtagagattctcctgcctcagcctcctaagtagctgggattacaggcgaccgccaccacgcccagctaatttttttttttttttttgtatttttagtagagacggggtttcaccatgttggccaggctggtctcgaactcctgaccttaggtgatccacccacctcggcctcccaaaatgctggaattacaggtgtgagccactgtgcctggctttgttggttttaacagttctttcccatgcaggctgcagctgaacagccaagtcccctccttgggtcacatatttttctgaaaatgttataaaaaaattgagtccactggcctgggctaattacctagcagaacatccccatggtttggtgattctgaatatcgctgccaaacaagcacttgtagaggctcaaacaaggccataaaacatggcaatgggggcgcgctcccactctgggaaatgaaaatctgacgatactttgaattacagtggatcaagattaattccaggctctacttagaggaagctttcaggcccagtggtttagacataaaagcagtttgccctaatgcggcaggtgaaagctgtgacaactctattgcttggtgccaattacatttatggacttgtacccaggagtgctaggaaattgtcaccattagtgctgacgtactgccagttgttggctctgtctagtggggttctgatttgaagactcattattaatattccctgtagtgatctgcaatgctgctccattatggcaagtctgtcaggaacggagtttgtgtaggaattttagaaaacagcaataggttgagggctatgtggtaggccccagagcttctcaaactactgtgcacacaaatcacccagggtctcgttgagatgcagattcggaatcacgtcctgagctgaggcttgatacttttcttcttttttggagacaggatctctctctgttgcccaggccagagtgcaatggtgcagtcatggctcactgcagcctcaaattcttaggctcaagcaatcctctcaccttgccttctgagtagttgggactacaggcgttagccactacgcctggcttttttttttttttgagatggagttttgctcttgttgcccaggctagagtgcaatggcatggtcttggctcactgcaacctctgcctcctgggttcaagtgattctcctgcctcagcctcccaagtagctgggattacaggcatgagccaccacacccggctaattttgtatttttagtagaggcagggtttcaccatgttggccaggctggtcttgaactcctgactttgggtgatccacccgcctcggcctcccaaagtgctgggatgacaggcatgagccaccatgcccggcacctcgcctggctttttaatttttgagatgtctggctctgttgcccaggctggagggcagtgttgcgatcttggctcactgcaaccttcgcctcccaggttcaagcgattctcctgcctcggcctcccaagtagctgggactgcaggcgcaaaccaccatgccagactaattggctgtttaatttttaatagagatggggtcttgctttgttgtccaggctggttgaactcctggccttaattgatcctcctgccttggcctcccaaagtatcgggattgcaggagtgagccaacatgctcagcctgatgttgcatttctaaccagcatccacgtgatgccacagatgctgctgctgctccagcgggaatgtgggaaaagcacaggctcaggagtcagatggacatgggtggacatgggctctaaacctgactctgcccttggttgctgtgtgatgttgggcaagttgctgaacctctctgaattttggatttctcatgtgcaaaatagggatcacttctgccttttaggttctttgaagatttataataacgtacatgcataggttttcttcttgctcccagaggggcagggtgaggtcactctcctgcatgctctcactacaggttcagctgagaccgtttttcttctctaaagtacttggctttcttcttccaagtcaggatttctccgcctcggcgctactcacattttgggctggatcattttgtgttgtgggggatgctccgtgattaccgcattatagaacgttcagcagcatctctggcctcacccactggatactggtggcacccgtctcccctacttgtgaccaccgaaaatgtctccaggcactgccaaatgttcctggaggcaaaatcactcacaaataggaaataatgacctaattagtaacttacattagcaattcattcaacaatatgtgttgagcatctactgtttgccagaccatacagcagggatgtagtgatatttaagacaaacaaggtccctgacctcatggagactttttcctttttggacctcagtcttctccgctgtaatgtgggtatcacaaggctgcggacctcctaaatttgttgggaagatgaagttagacttgcaagtgcctggcccctggcatgagggattagccaatgccaggggtatgatgggcctagggatggaacctgggagcttggggagaagcgagtgtgggcagggacagtgcatggagaagccaggaaacctgagctgcaagggaggcggaaaggggccatgaaaggccctggtgcaaagtgtgcggcagcagcaaggcaggggaaaggggctgcagggagggccaagggtagcaggaagatgggaccaaaactggagagaaggagagagacagtgggacatagaggatgacaggaaggggtggagatgggaggagagaggcacagatggagaagataaaaaaccagacagacagacatgtacacacgtgataagacagagagaccaaggggcggagggaaaatgagtccaggcggaagggaacacctctgaggaagatcactgcacaaaccctggtcagctgcacatgaccccaaagagtggctcttaggtttattccaaacgtacctgatttgggtgataaagagttaaaattaaatacaaaggccaatgccagtccattcctggcgccagctcctgcctcttccttctcatggggccctcaccagagtgatggggtggagcatacccaaccctgggaggaaatgaggcttttgtgccgagcggcaatatgatggcaatactggcagtggtagtcaacccatctgtaaacagctgacagagggcagtacaagaatccacctcacagccagggccgcaaccgcaagtaaagcacacagctgaaatgactgacgtgggtggaactgagctgagaaggaacgtggctcggcttgaccctggagcacacatcacaaccatgagaaacaggcaactaaagtgacctccagcccacagcaacaaccttctctggctacaactgggaggcagggacagaccccagaaaaccatcttgggtcatctaaggtacgtgtaaccatatttttaaaatgacaaaatctcaagcatgttgctttggtgagcttctgattttactagaaatacactctaagaacagtcgagacgccgcgccttgtggaggcgatgggtcatgttactggttctgcgatgatcttccagagctcctcttctccaccgacagtatggctgtgcaggcatttttcaatctgtgggcgagtcgggagagcgttttaaacacagcatcagtcaagtcgtcgtcgtaaaacacttcggctgcaaacaggatggtggtgtgatcgtacaagtcagaaatttcctcttgtgaccaactgaaggggaccttgggatctgtgcagaggtcgtccttcagccagtccagttctttgaccctaactataccacctgtgagtgagtcctggccgtgctggatgcagggctggaaaggagactgtcaggaggaggcaaggagagcaggccggggctgggccagggaggcctgggaattcaaggagctcagacttcaccccacaggtgatgacgcccctgggaggttttcagcagcaagtgaagtggactggcttgcatctgagaaagggcactctggatgtttcatgaggacatcttggacgggtcaactaaggagctggggagaccagctcaggggccgccgccagtgtccgggagagaaagagctggagtaggatgacgcagtggatctccagtggcagccaggtggctgttgagggcaatgtttcgctggcacatggacaagagatctgcaccgacatctgtacaataaacggtccgtgccatggtggctgcgatgatgctagcgagccccgtgccggccccgagctccagcgctgtacatcctcggaagaggtcctgtcggaacaggatgtagtctgccaggagcagggcgccccgccacacctattctgatgatatcgtgcgggctgccttgtgcttcctctcccaggacgtcgtcttcttcctgtgctagaatcatgggatgtaccttgtctctcagaggccctgctgggttggaatcagaggcggctcgtggtcttctcaccacgtccaaatccccatcctcatccagctgagcttcagccacttcctggccagtggtgtcagtcccggcctggagggagaaaccctcattaccatggccacttcctggaggggaccctgtgctgcctgtctcagcagaaggaggctcctttgtgtgaacatctctgtgactgccacccttggctcctgaatctgtccaagagtcttggctccatagaagcttgaattgggacaggaaaactggctgccccacgctgttcagccgtaccatgagatgtctatggttcggggtatagaggtggacatctgacagcacagtgtcgctcctaaaggtgacctcgtccatggctgccgcaggagccagctgtaccatggcccaggctccaccttagtcctaggacaggagtccctcagaggtgagaatgggtcctcagcatggcaggtcccagaggagatactgcagacaggtccaagctggtagcgagtagctttgcatcgccctgggagaagatctcagagacttggccagggaagagaatccagccgccgcggggcccagcctgggatcccacccgactcccgtctctgtgggacttaggcggccgccataacaggcggtctgcgcaggcgcggccccgcccccgcgtgc

SEQ ID NO: 11342 - RNA, 6774 nt, Homo sapiens
  source 1..6774: mol_type = other RNA
ctgaatagctgggactacaggtgcccgccaccacgcctggctaattttttgtatttttagtagagacggggtttcaccatgttagccaggatggtcttgatttcctgacctcatgatctgcccacctcggcctcccaaagtgctgggattacaggtatgagccactgcgcctggcccatttagtatgatctttacaataattctgtgaagaaagaattcttaccctctttttttcccatttatttatttatattattttttgagacggagtctcgctctgtcacccaggctggagtgcaatggtgcaatcttagctcactgcaaactccacctctcaggttccaattctcctgcctcagcctccagagtagctggaattacaggcacgccaccatgcccagctatttttttgtatttttagtagatacggggttttgtcatgttggccagactggtcttgaactcctgacctcaggtgatccatttgccttggcctcccaaagtgccgggattacacgcatgagccacatctggctttttttcatttattgataaatgaaattttgcatattatggggtgcatatgaatgtgttttatatacacagaatgtgtaattatcaagccagggtatttgaggtattcaccaccttgagaatttataattttatgtgttgggaacatttcaagttctctcttctagcaactttgaaatacacaatatattgttgctaactgtagccaccctagtctgctaccaaacattagaaggtatttcttccctaagtttgtacccattcaccaacctatcaagaagttttactattttacaggtgaggaaactcaggttcagagaggctaggtcatttgtccaaggtcattgctgttacacagcagaggcaggatttaaaccctggcttgctcaactccggagttggtgggtttttttttctttagaaatagcgtctctgtctgtaaggctgtgagggtgtagtgcagtggcacaatcacagttcactgcagcctagaattccttcgcttaggcgatgctcccgacccagcctcctgagtagctgggagtacaggtgcatgacacacctggctaattaaaaaaaagttttttagagatagggtctctgtatgttgcccaggctgatctcaaactcctgtcctcaagtaatcctcctgcctttgcctcccaaagtgctgggatcacaggtatgagccaccacatccaacccagagtttgtgctcttaaccagggatgacatgttgcaacttcactcctcacagtgtggcccacagacgagcatcatcagcatcacccgggagcttgttaaactgcagcatcaggccacatccagggcctgagtcagaatctgtattttgacaagatcccaagtgattcgtgtgcatactagtttgagaagctttggggaccacagtttcactaatggttttttttttttaatttcttttgagacggagtttcattcttgttgcccagggtagagtgcaatggcgcagtcttggctcactgcaacctccacctcccgggttgtagagattctcctgcctcagcctcctaagtagctgggattacaggcgaccgccaccacgcccagctaatttttttttttttttttgtatttttagtagagacggggtttcaccatgttggccaggctggtctcgaactcctgaccttaggtgatccacccacctcggcctcccaaaatgctggaattacaggtgtgagccactgtgcctggctttgttggttttaacagttctttcccatgcaggctgcagctgaacagccaagtcccctccttgggtcacatatttttctgaaaatgttataaaaaaattgagtccactggcctgggctaattacctagcagaacatccccatggtttggtgattctgaatatcgctgccaaacaagcacttgtagaggctcaaacaaggccataaaacatggcaatgggggcgcgctcccactctgggaaatgaaaatctgacgatactttgaattacagtggatcaagattaattccaggctctacttagaggaagctttcaggcccagtggtttagacataaaagcagtttgccctaatgcggcaggtgaaagctgtgacaactctattgcttggtgccaattacatttatggacttgtacccaggagtgctaggaaattgtcaccattagtgctgacgtactgccagttgttggctctgtctagtggggttctgatttgaagactcattattaatattccctgtagtgatctgcaatgctgctccattatggcaagtctgtcaggaacggagtttgtgtaggaattttagaaaacagcaataggttgagggctatgtggtaggccccagagcttctcaaactactgtgcacacaaatcacccagggtctcgttgagatgcagattcggaatcacgtcctgagctgaggcttgatacttttcttcttttttggagacaggatctctctctgttgcccaggccagagtgcaatggtgcagtcatggctcactgcagcctcaaattcttaggctcaagcaatcctctcaccttgccttctgagtagttgggactacaggcgttagccactacgcctggcttttttttttttttgagatggagttttgctcttgttgcccaggctagagtgcaatggcatggtcttggctcactgcaacctctgcctcctgggttcaagtgattctcctgcctcagcctcccaagtagctgggattacaggcatgagccaccacacccggctaattttgtatttttagtagaggcagggtttcaccatgttggccaggctggtcttgaactcctgactttgggtgatccacccgcctcggcctcccaaagtgctgggatgacaggcatgagccaccatgcccggcacctcgcctggctttttaatttttgagatgtctggctctgttgcccaggctggagggcagtgttgcgatcttggctcactgcaaccttcgcctcccaggttcaagcgattctcctgcctcggcctcccaagtagctgggactgcaggcgcaaaccaccatgccagactaattggctgtttaatttttaatagagatggggtcttgctttgttgtccaggctggttgaactcctggccttaattgatcctcctgccttggcctcccaaagtatcgggattgcaggagtgagccaacatgctcagcctgatgttgcatttctaaccagcatccacgtgatgccacagatgctgctgctgctccagcgggaatgtgggaaaagcacaggctcaggagtcagatggacatgggtggacatgggctctaaacctgactctgcccttggttgctgtgtgatgttgggcaagttgctgaacctctctgaattttggatttctcatgtgcaaaatagggatcacttctgccttttaggttctttgaagatttataataacgtacatgcataggttttcttcttgctcccagaggggcagggtgaggtcactctcctgcatgctctcactacaggttcagctgagaccgtttttcttctctaaagtacttggctttcttcttccaagtcaggatttctccgcctcggcgctactcacattttgggctggatcattttgtgttgtgggggatgctccgtgattaccgcattatagaacgttcagcagcatctctggcctcacccactggatactggtggcacccgtctcccctacttgtgaccaccgaaaatgtctccaggcactgccaaatgttcctggaggcaaaatcactcacaaataggaaataatgacctaattagtaacttacattagcaattcattcaacaatatgtgttgagcatctactgtttgccagaccatacagcagggatgtagtgatatttaagacaaacaaggtccctgacctcatggagactttttcctttttggacctcagtcttctccgctgtaatgtgggtatcacaaggctgcggacctcctaaatttgttgggaagatgaagttagacttgcaagtgcctggcccctggcatgagggattagccaatgccaggggtatgatgggcctagggatggaacctgggagcttggggagaagcgagtgtgggcagggacagtgcatggagaagccaggaaacctgagctgcaagggaggcggaaaggggccatgaaaggccctggtgcaaagtgtgcggcagcagcaaggcaggggaaaggggctgcagggagggccaagggtagcaggaagatgggaccaaaactggagagaaggagagagacagtgggacatagaggatgacaggaaggggtggagatgggaggagagaggcacagatggagaagataaaaaaccagacagacagacatgtacacacgtgataagacagagagaccaaggggcggagggaaaatgagtccaggcggaagggaacacctctgaggaagatcactgcacaaaccctggtcagctgcacatgaccccaaagagtggctcttaggtttattccaaacgtacctgatttgggtgataaagagttaaaattaaatacaaaggccaatgccagtccattcctggcgccagctcctgcctcttccttctcatggggccctcaccagagtgatggggtggagcatacccaaccctgggaggaaatgaggcttttgtgccgagcggcaatatgatggcaatactggcagtggtagtcaacccatctgtaaacagctgacagagggcagtacaagaatccacctcacagccagggccgcaaccgcaagtaaagcacacagctgaaatgactgacgtgggtggaactgagctgagaaggaacgtggctcggcttgaccctggagcacacatcacaaccatgagaaacaggcaactaaagtgacctccagcccacagcaacaaccttctctggctacaactgggaggcagggacagaccccagaaaaccatcttgggtcatctaaggtacgtgtaaccatatttttaaaatgacaaaatctcaagcatgttgctttggtgagcttctgattttactagaaatacactctaagaacagtcgagacgccgcgccttgtggaggcgatgggtcatgttactggttctgcgatgatcttccagagctcctcttctccaccgacagtatggctgtgcaggcatttttcaatctgtgggcgagtcgggagagcgttttaaacacagcatcagtcaagtcgtcgtcgtaaaacacttcggctgcaaacaggatggtggtgtgatcgtacaagtcagaaatttcctcttgtgaccaactgaaggggaccttgggatctgtgcagaggtcgtccttcagccagtccagttctttgaccctaactataccacctgtgagtgagtcctggccgtgctggatgcagggctggaaaggagactgtcaggaggaggcaaggagagcaggccggggctgggccagggaggcctgggaattcaaggagctcagacttcaccccacaggtgatgacgcccctgggaggttttcagcagcaagtgaagtggactggcttgcatctgagaaagggcactctggatgtttcatgaggacatcttggacgggtcaactaaggagctggggagaccagctcaggggccgccgccagtgtccgggagagaaagagctggagtaggatgacgcagtggatctccagtggcagccaggtggctgttgagggcaatgtttcgctggcacatggacaagagatctgcaccgacatctgtacaataaacggtccgtgccatggtggctgcgatgatgctagcgagccccgtgccggccccgagctccagcgctgtacatcctcggaagaggtcctgtcggaacaggatgtagtctgccaggagcagggcgccccgccacacctgcttgccaacatcctccaggggcgtggccatggtgtgctctattctgatgatatcgtgcgggctgccttgtgcttcctctcccaggacgtcgtcttcttcctgtgctagaatcatgggatgtaccttgtctctcagaggccctgctgggttggaatcagaggcggctcgtggtcttctcaccacgtccaaatccccatcctcatccagctgagcttcagccacttcctggccagtggtgtcagtcccggcctggagggagaaaccctcattaccatggccacttcctggaggggaccctgtgctgcctgtctcagcagaaggaggctcctttgtgtgaacatctctgtgactgccacccttggctcctgaatctgtccaagagtcttggctccatagaagcttgaattgggacaggaaaactggctgccccacgctgttcagccgtaccatgagatgtctatggttcggggtatagaggtggacatctgacagcacagtgtcgctcctaaaggtgacctcgtccatggctgccgcaggagccagctgtaccatggcccaggctccaccttagtcctaggacaggagtccctcagaggtgagaatgggtcctcagcatggcaggtcccagaggagatactgcagacaggtccaagctggtagcgagtagctttgcatcgccctgggagaagatctcagagacttggccagggaagagaatccagccgccgcggggcccagcctgggatcccacccgactcccgtctctgtgggacttaggcggccgccataacaggcggtctgcgcaggcgcggccccgcccccgcgtgc

SEQ ID NO: 11343 - RNA, 1250 nt, Homo sapiens
  source 1..1250: mol_type = other RNA
ctgaatagctgggactacaggtgcccgccaccacgcctggctaattttttgtatttttgtagagatggggtttcaccgtggtagccaggatggtcttgatctcctgacctcttgatccgcccgcctcggcctcccgaagtgctgggattacaggcgtgagccaccgcgcctggcctgagttcctccttctctaattgcctaagcacaggttggtggaaatgctgggaggggattcaagcagctgacagcagagattccaggtgacacagctccagtttcttcaaagagtcttgaatccatcaggaatgcttttgatcacaagtaacgaaacagctgaccaacaggcaccaggcagtgaagagaggccgtcagctcacacggtcagaagtccggaggtgggcggtcccagctggcataggtgcaggaggatgggtgtcagcaccaggcttcctggttacctgctctgccacccacagcacacggctgtccatgccaagcctgtcacctcatggtcacaagatgccaccatgttccaagtatcacatcatcacacagaagcgttggaggcaggaagttggggaaggtgcagaaaggtcttttccttacatgcctttgtcttgtatctgaagaaaaataaaagtatttcctggaagccccatcagcaggcttgctctgtgtctcgctggccacagctgggttgtatgccaagtctgtgccatcataggtcagtgcatactgtggtaagctcagggagatggactctttctgatctgggggtccaagcaggcttactcagctggttaatcacagagctctggttggggcatccggcccccgactcatcagcatcggctggctgctcgtcccctggaatggctcctaatcccctcggcagtgactaagcaccttccagtcactgctccagtcattaatttcagcacgggcgcggcctggccgtgctgttctcctggagcgccaaggctgtccgcgcagccattgatttaggagacaatatcacttgcttccaagtttatgaggcagtaaacagcccccgcatagtgatgaatgccgaggtgtttgctcagcacatttgctgtgcgcatttattacaagggctgtgctttaaagcaaatgaaactgcaactattttcatttcctccggtggggccggcccctcccccagcggttgtcctatctatttgatcctggatccctcttccctgggtactgggctgcaaccctgtgaccag

SEQ ID NO: 11344 - RNA, 667 nt, Homo sapiens
  source 1..667: mol_type = other RNA
ctgaatagctgggactacaggtgcccgccaccaggaatcttcacactcaggcttgaaactccatgatcatgaagttcatcctcaaaaaggagaacttcttcaaaaaacttaatctgttctctggctttcaatttttctgtatctatatgatctgttgtaggtacaacctttaacttaagagattctccaagtaaggttcccttataatctgttgtataggtccaatcatatggtttaataacctctttggagtgttcaccctccgtcctgctttcttgccactcttcagcacaggccactttaagcattccttggtagttgtttacacatcttaacgcatctgtagcattgaactcaattccaaagccagacccatgctggattcttaaaacgttgtctccaaacatcatttcagggagagatggcatatgtaattcatcggctaatttctccacatccgccgacttcatgatgtgggtcttggacgccgtcagcttccagggcccgaagcagaaatcccggtggctgctctggaagccgtggatcatcatggctgaggcaggacccgcagaggccacaaggaataagctgaagcagcggcggcggcgaacaccggttcctccgcctccctccggcccagcctcctaggcttccgagccgttaccat

SEQ ID NO: 11345 - RNA, 6774 nt, Homo sapiens
  source 1..6774: mol_type = other RNA
ctgaatagctgggactacaggtgcccgccaccaggcccggctaattttttgtttgtttttttagtagagacggggtttcactatgttagccaggatggtctcgatctcctgatctcgtgatctgcccgcctcggcctcccaaagtgctgggattacaggtgtgagccaccgcacctggccccgagatttttaaataagttttgaacatgaataaaaatatggtgctcacatttattactttaaagaaagagactcgtctatcaaaaatttgatacaagtttttcacttattttcaaacatctactagaataattttcattcttccaggtgttcaaagtgcccaagcaggatgtaggttagttctacccttaaacttaaggtgtagattataagcacgttttccatttgcaacacaacagtaggcattcttgttaaattagtttgagaaatttgttttattttgtacaaggtacaatccctctgcacagtgaacatatattacaaatctgtgatttaaaaaagtattgccgtttcatagtctcattaatacctctgtacaataatggtttttctttcattcattttaattgtacacatattaattttttgaaaatttagtttctgaaaaataattgaacagatctttcaaagtcacccataaaatgcacagtatacatgtttaggctgaccatgaacctatttgtgatggtgttagacagaagtttctaacagttgctttgtaagattgaaatgtcttttactgataactgttcgataggggaaggcagctattgtcaccataatcacaccctctgcctttcccttctcctctgtattgcctggtttgacttgtattacatttccttaaaaagtcatggactgctagagctgaagggttagtagagctgtcttcccactctctgcttctcccctttttatgcataggaaaaaagggagcccagagagggcgactaacttgaccagagtaacactgaaatctcttgattcagtgtctagccattccacctcttgctgaatacctttgcccagaggatagttgacaaaagcggcgaaacttcaaacttgagtgatgctgcttgtttgcagtttgccaggcagcagttattgtacatgcaggataagggaagaagagaaaacctgggattgagttgaagtttctccttgctgatctgacatcttcatgctgctcatccttgcttcacaaacacttgctgccctgaaatactgaggtaagctgcttacctatatttctttctacatatgtatgagaaatatttacttgggtctccaaagtaattttctaatatttatattttaataaggcttttttggaaagtaaatttactattgctactcagttgctcccatgcacacatgcaacattcatgtaagtattacatattttcctctaacagtaaaatctgcttatgccttgagtgatgtgggaaggggagatgtactcatttatttatttttttgctttttctgattattgcccaaagtattgtgttccatggcaggcttccagtttctatcaagggtttcagaactctcatacttcctgtagcagtattccagcttcgcagtcatttagttcctcttctgtgtatctttttggaagtgttttttactggctggactgtaccagtgaatagagtggtacaggagtagccgttagcttcctaggtttgccctttttgtttttaattcttgtgagaaggttctctttagggcttgggagttgatttcatttcatttggacttatctgagcctcagtttatctgtgttcatagtggaaggtatagacacatctgaatactgggatctggagcattagctcattgtaatgcatattgggctagctcagtaagtagtagttttaagatagaaggtggaaggacttcatatcctcatgctgtttacagtaacgtttttacatcacgttacagcaactggttacagtccattctttttttgatcatttagttccattaaaaagcataatgtactttaagcagtgtaaacttgctgtatccacatttgtccaatttcctgtatacttttaggtttcatactacgtcaatctcaagatttatgaagaacttgaaagcaagtactcttgagtcaagggatgctgaccaaataaaatgaggaggccaactagccgtcttttacttaatcccgaccagtctatgactgcttgcttaaaggatcatcttagagctctgttttacatggaatgattcaggtgtcggatggactaagtagatatgacaaagccaggactaacttgtaatgtccttgaactttgaattggcaaaatttgataaagctgccctaggaatcttattgtagactgaaagagacactgctgcactttggaaacgtgtgtgtgtgtctctgtgtgtttaaacctatcacttagggggcagaagaaagtaaagtcttgttttttaaaatagaagttgtcagcattagactatatagattctgtaatcttggctgttgtaatttgatggaccagacagatatgtacagacattttaagactgttctgtttaagaacagttcatgtctgtgtactaattgtcttcggtaataaaacagatgttgatggtaacagcaaccaaaagtacatatacgtttcaggtgctttaaagtaatcctcttccctccccagtctcctttttgtcctaggaaggtttgttaaacctacatgtttttaaaatatcacgtttcagataaatatatatatatatatcagctatatttagctgatgttgatgagtagctgtatcttaaaatgttttaaaaatcatataatccagggcatttggggctgagtgggtgataggatttgcctttgagaacacaattccttgaacaattatcccagtcccacctggacgctcttctttagttccaggtgaacgtaataactaacatgcagctggagccagtctgtaccattacttcaagtcaagggactgtcttctttcagagtcagaatattcagtagagcacactgcaagagagaagcttatccctcttaagattgcttgtcctgggacggcccattggcagggctctgtcttactgggaggaggtcataatgaccaggaatatggctgttcctaggtaggtcgtatgcattctggatatagctggagttatgaccgcaaccttcttggaccacactgactgtgggctcaacttcatatatatttttattagatgtcgacaaggatggcacatctgtgtacggagaccccatgtgcacaggcgacttcatttctacatagctgctttctggaagcttgcaggtgaggatgggtgggtccttaattgtggcgtaagggttttcactgctattcaaggaacaagtactagaactgcacacggattctttcatgtaatctttgaagcctttgtccataatgtatgtgttctgacgtctatccattccacaagcacctgagagggagtagtcggtgctggtcatcctcatggcaggtgtgtaggagacacggggagccaggtctcggcccttctctttctgccgccgccgatgccaggcaaataggcccagcagcaccacaatgaggaataacaggagcatgatgcctgtgacagcacccaccgagtgccgctctgcacccagtgctgggctgatcttggtgtagggattcagctcctccatcatgagggcagcttggtcacacctgattcctttgaagccagggctgcagtaacaggtgccggtgacatggtcacaggtggagttgttcatgcactcacatagctgctgacacccatagccaaaggttcctggggcacatctctgctcacagtgttgcccggtgaagcctgtgcggcaggtgcacttgccactgatgtggtcacagctggcgccattctgacactggcatacgcgcccacagtccttcccaaaaaatgctgctgggcagcgctgtgtgcagaagagtccagtccagccaggggtgcagtggcaggccccgtcctcggcgctgcagctcgccccgttgtggcagctgcatgcgtggaagcaggcggggccccagaacccgggtgggcaagcctgtgagcagtccttgccaatccatccaggaaagcactggcaggagccatcgatagggctgcaggtcccgttgttggcacaggagcagagctgggcacagtcctgcccaaagtatcctccagcacacacttggttgcagagagctccagagaatcctgggaggcactcacagatgccgctgatgtggtggcagggcctgctgctgtgcacgcagagggggcatggctgggcgcagccgtggccatagaacccaggggggcagattctctggcataagggtcctcggaagccaggggcacactcgcagctcccatcctctggggagcaggagcctccattctcacagctgcaggagacagagcagttggggccccagcggccaggtggacacgtgctgtcacagcggatgcctgtccatccggccaggcagcagcagtggcctgtgacggggtcacatccatcagcatggctgcagtcacagtgttcactgcagttcagcccaaatgtgccatccgggcaaggcagctcacaggtgtctcccagccagccaggagtgcaggagcaggagccgtctatggggctgcaggctgccccattggcacaggtgcagctctcgttgcagttcaggccccacgtcccactgggacatggcagggtgcagtccaggccctgccacccttccttgcaggtacaggagccatctactggggagcaggtgccaccattgttacagctacagatggacgagcagttggggccataggtccctgctgcacaggaaacggcacagacctctcccatgaagcccggagcacaagtgcagcccccagtgatgctgtggcagtcggcgccattctgacaggtgcaaggcagctggcagccatcgccatagtagccaacagggcaggattcattgcagtggtgaccagaccagcctggctggcaggtacaagctccagttactgggtggcagctgatggtgttgtcagcgtcacaggggcagggcagggtgcagcctgggccatgcaggccctccgggcacagtcgctcctggcagcgtgggcccttgtagccaggctcacactcgcaggcacccgtggtgggtgaacactgccccccattgtggcagtcacagtgctgtgagcactggaagccgaaggacccgaaggggcactcctcttggcacctgtcccccatgtatccagctgtacagtggcactgtccagtcacgtggtcacactgccctccatggtggcaaggacaatcctggctgcagttctggccaaatgtccctggtgggcagggctgggcacacactgctcccgtccagcctggggggcaggcacactcgccagtgatgtggtggcaggtgcccccattctgacaggggcagcgcagctcacagtgagctccatggctcccaggagggcacagctcctcgcagtagacgccggtgtagccaggtgcgcagaggcactcgccggcgcgggggtcgcagctggcaccgtgtcggcactggcacggcagctggcatcccttgccgtgggtgccaggtgcgcagagctcctcgcagcgccatccacggaagccggcggcgcacacgcaggcgcctgtgatggggttacacagggcgccgttctggcactggcaccggttgctgcagtggggcccccagtggtcgctgtcgcagccgctggagcagtcgggccctccccagccaggctcgcagtggcaggtgtccggggaaacgcagcggccgtgcacacactcctccgtacacaggggtatgcagaagtctccgctctcatagtagccagggcagcactgggacctccgccggtacatggtccggaggcctctccgatacgccgtcttataactgatccggtgcctggtgcacttgaaccagttgaggatgtctgtgcatcgtgtgtaatagatctgatcgaaggggtgtgcatacgattcctggacagtcacagcatagctctcccagtggctgcacacgttggggtcctcggggttcagggcaagggtggcttgcaggaaggagaaggcaatgagccccgtcagggagagcaccatcccgggccctgcacaggagaacaaaggaggctgcgtctgtgatcagaccatgttcctggcaactacttagtttcccatcgtcgtgggtaatgagcatttgatatttcacattgcaggctttgactaacactgtaacagttcactggttctgagtaacaggagagtgggaagcctgagtcaggaaaaagtccaaattctaggccaggggttctgaatgttttttgactcagggactgctctgagaatccagtgaaaggtatagatgttctctccaggaaaatgcccacaagtgcaaaatcggctataattgcagggtgtcctcaggcccccgggcccatccttggacccagggaccccagatctggactgctttaaagggaatgccctccccattcccttatccctcatcattgacattctttgcccatctacttcctttccctactccctcctgccaaggagaaagagaaaaaagatgtctggtgtggacctggggggaaatgagccaagaaaaccctgagctctgggcccacaagccatggaagactggatcttgcttcttctgtct

SEQ ID NO: 11346 - RNA, 6926 nt, Homo sapiens
  source 1..6926: mol_type = other RNA
ctgaatagctgggactacaggtgcccgccaccaggcccggctaattttttgtttgtttttttagtagagacggggtttcactatgttagccaggatggtctcgatctcctgatctcgtgatctgcccgcctcggcctcccaaagtgctgggattacaggtgtgagccaccgcacctggccccgagatttttaaataagttttgaacatgaataaaaatatggtgctcacatttattactttaaagaaagagactcgtctatcaaaaatttgatacaagtttttcacttattttcaaacatctactagaataattttcattcttccaggtgttcaaagtgcccaagcaggatgtaggttagttctacccttaaacttaaggtgtagattataagcacgttttccatttgcaacacaacagtaggcattcttgttaaattagtttgagaaatttgttttattttgtacaaggtacaatccctctgcacagtgaacatatattacaaatctgtgatttaaaaaagtattgccgtttcatagtctcattaatacctctgtacaataatggtttttctttcattcattttaattgtacacatattaattttttgaaaatttagtttctgaaaaataattgaacagatctttcaaagtcacccataaaatgcacagtatacatgtttaggctgaccatgaacctatttgtgatggtgttagacagaagtttctaacagttgctttgtaagattgaaatgtcttttactgataactgttcgataggggaaggcagctattgtcaccataatcacaccctctgcctttcccttctcctctgtattgcctggtttgacttgtattacatttccttaaaaagtcatggactgctagagctgaagggttagtagagctgtcttcccactctctgcttctcccctttttatgcataggaaaaaagggagcccagagagggcgactaacttgaccagagtaacactgaaatctcttgattcagtgtctagccattccacctcttgctgaatacctttgcccagaggatagttgacaaaagcggcgaaacttcaaacttgagtgatgctgcttgtttgcagtttgccaggcagcagttattgtacatgcaggataagggaagaagagaaaacctgggattgagttgaagtttctccttgctgatctgacatcttcatgctgctcatccttgcttcacaaacacttgctgccctgaaatactgaggtaagctgcttacctatatttctttctacatatgtatgagaaatatttacttgggtctccaaagtaattttctaatatttatattttaataaggcttttttggaaagtaaatttactattgctactcagttgctcccatgcacacatgcaacattcatgtaagtattacatattttcctctaacagtaaaatctgcttatgccttgagtgatgtgggaaggggagatgtactcatttatttatttttttgctttttctgattattgcccaaagtattgtgttccatggcaggcttccagtttctatcaagggtttcagaactctcatacttcctgtagcagtattccagcttcgcagtcatttagttcctcttctgtgtatctttttggaagtgttttttactggctggactgtaccagtgaatagagtggtacaggagtagccgttagcttcctaggtttgccctttttgtttttaattcttgtgagaaggttctctttagggcttgggagttgatttcatttcatttggacttatctgagcctcagtttatctgtgttcatagtggaaggtatagacacatctgaatactgggatctggagcattagctcattgtaatgcatattgggctagctcagtaagtagtagttttaagatagaaggtggaaggacttcatatcctcatgctgtttacagtaacgtttttacatcacgttacagcaactggttacagtccattctttttttgatcatttagttccattaaaaagcataatgtactttaagcagtgtaaacttgctgtatccacatttgtccaatttcctgtatacttttaggtttcatactacgtcaatctcaagatttatgaagaacttgaaagcaagtactcttgagtcaagggatgctgaccaaataaaatgaggaggccaactagccgtcttttacttaatcccgaccagtctatgactgcttgcttaaaggatcatcttagagctctgttttacatggaatgattcaggtgtcggatggactaagtagatatgacaaagccaggactaacttgtaatgtccttgaactttgaattggcaaaatttgataaagctgccctaggaatcttattgtagactgaaagagacactgctgcactttggaaacgtgtgtgtgtgtctctgtgtgtttaaacctatcacttagggggcagaagaaagtaaagtcttgttttttaaaatagaagttgtcagcattagactatatagattctgtaatcttggctgttgtaatttgatggaccagacagatatgtacagacattttaagactgttctgtttaagaacagttcatgtctgtgtactaattgtcttcggtaataaaacagatgttgatggtaacagcaaccaaaagtacatatacgtttcaggtgctttaaagtaatcctcttccctccccagtctcctttttgtcctaggaaggtttgttaaacctacatgtttttaaaatatcacgtttcagataaatatatatatatatatcagctatatttagctgatgttgatgagtagctgtatcttaaaatgttttaaaaatcatataatccagggcatttggggctgagtgggtgataggatttgcctttgagaacacaattccttgaacaattatcccagtcccacctggacgctcttctttagttccaggtgaacgtaataactaacatgcagctggagccagtctgtaccattacttcaagtcaagggactgtcttctttcagagtcagaatattcagtagagcacactgcaagagagaagcttatccctcttaagattgcttgtcctgggacggcccattggcagggctctgtcttactgggaggaggtcataatgaccaggaatatggctgttcctaggtaggtcgtatgcattctggatatagctggagttatgaccgcaaccttcttggaccacactgactgtgggctcaacttcatatatatttttattagatgtcgacaaggatggcacatctgtgtacggagaccccatgtgcacaggcgacttcatttctacatagctgctttctggaagcttgcaggtgaggatgggtgggtccttaattgtggcgtaagggttttcactgctattcaaggaacaagtactagaactgcacacggattctttcatgtaatctttgaagcctttgtccataatgtatgtgttctgacgtctatccattccacaagcacctggtgagtgtggctcagcggggcggctgaggtgtctaagttcaatgtagaagtcctcgggcgggtacctggcctccagggcactgatctggaaatgggagtctaacacgttcacatagctgtagggggtccagcctgctgtgtctctgtcaagggacttgttactgagcttggtggggctgttcctgtccagagtgctggcctggctggtggcaggccccccacatgccagtgcgtggtagctggaattggaaaagcagtgggcatggctgctactttgagacaaatctgagagggagtagtcggtgctggtcatcctcatggcaggtgtgtaggagacacggggagccaggtctcggcccttctctttctgccgccgccgatgccaggcaaataggcccagcagcaccacaatgaggaataacaggagcatgatgcctgtgacagcacccaccgagtgccgctctgcacccagtgctgggctgatcttggtgtagggattcagctcctccatcatgagggcagcttggtcacacctgattcctttgaagccagggctgcagtaacaggtgccggtgacatggtcacaggtggagttgttcatgcactcacatagctgctgacacccatagccaaaggttcctggggcacatctctgctcacagtgttgcccggtgaagcctgtgcggcaggtgcacttgccactgatgtggtcacagctggcgccattctgacactggcatacgcgcccacagtccttcccaaaaaatgctgctgggcagccctgtgagcagtccttgccaatccatccaggaaagcactggcaggagccatcgatagggctgcaggtcccgttgttggcacaggagcagagctgggcacagtcctgcccaaagtatcctccagcacacacttggttgcagagagctccagagaatcctgggaggcactcacagatgccgctgatgtggtggcagggcctgctgctgtgcacgcagagggggcatggctgggcgcagccgtggccatagaacccaggggggcagattctctggcataagggtcctcggaagccaggggcacactcgcagctcccatcctctggggagcaggagcctccattctcacagctgcaggagacagagcagttggggccccagcggccaggtggacacgtgctgtcacagcggatgcctgtccatccggccaggcagcagcagtggcctgtgacggggtcacatccatcagcatggctgcagtcacagtgttcactgcagttcagcccaaatgtgccatccgggcaaggcagctcacaggtgtctcccagccagccaggagtgcaggagcaggagccgtctatggggctgcaggctgccccattggcacaggtgcagctctcgttgcagttcaggccccacgtcccactgggacatggcagggtgcagtccaggccctgccacccttccttgcaggtacaggagccatctactggggagcaggtgccaccattgttacagctacagatggacgagcagttggggccataggtccctgctgcacaggaaacggcacagacctctcccatgaagcccggagcacaagtgcagcccccagtgatgctgtggcagtcggcgccattctgacaggtgcaaggcagctggcagccatcgccatagtagccaacagggcaggattcattgcagtggtgaccagaccagcctggctggcaggtacaagctccagttactgggtggcagctgatggtgttgtcagcgtcacaggggcagggcagggtgcagcctgggccatgcaggccctccgggcacagtcgctcctggcagcgtgggcccttgtagccaggctcacactcgcaggcacccgtggtgggtgaacactgccccccattgtggcagtcacagtgctgtgagcactggaagccgaaggacccgaaggggcactcctcttggcacctgtcccccatgtatccagctgtacagtggcactgtccagtcacgtggtcacactgccctccatggtggcaaggacaatcctggctgcagttctggccaaatgtccctggtgggcagggctgggcacacactgctcccgtccagcctggggggcaggcacactcgccagtgatgtggtggcaggtgcccccattctgacaggggcagcgcagctcacagtgagctccatggctcccaggagggcacagctcctcgcagtagacgccggtgtagccaggtgcgcagaggcactcgccggcgcgggggtcgcagctggcaccgtgtcggcactggcacggcagctggcatcccttgccgtgggtgccaggtgcgcagagctcctcgcagcgccatccacggaagccggcggcgcacacgcaggcgcctgtgatggggttacacagggcgccgttctggcactggcaccggttgctgcagtggggcccccagtggtcgctgtcgcagccgctggagcagtcgggccctccccagccaggctcgcagtggcaggtgtccggggaaacgcagcggccgtgcacacactcctccgtacacaggggtatgcagaagtctccgctctcatagtagccagggcagcactgggacctccgccggtacatggtccggaggcctctccgatacgccgtcttataactgatccggtgcctggtgcacttgaaccagttgaggatgtctgtgcatcgtgtgtaatagatctgatcgaaggggtgtgcatacgattcctggacagtcacagcatagctctcccagtggctgcacacgttggggtcctcggggttcagggcaagggtggcttgcaggaaggagaaggcaatgagccccgtcagggagagcaccatcccgggccctgcacaggagaacaaaggaggctgcgtctgtgatcagaccatgttcctggcaactacttagtttcccatcgtcgtgggtaatgagcatttgatatttcacattgcaggctttgactaacactgtaacagttcactggttctgagtaacaggagagtgggaagcctgagtcaggaaaaagtccaaattctaggccaggggttctgaatgttttttgactcagggactgctctgagaatccagtgaaaggtatagatgttctctccaggaaaatgcccacaagtgcaaaatcggctataattgcagggtgtcctcaggcccccgggcccatccttggacccagggaccccagatctggactgctttaaagggaatgccctccccattcccttatccctcatcattgacattctttgcccatctacttcctttccctactccctcctgccaaggagaaagagaaaaaagatgtctggtgtggacctggggggaaatgagccaagaaaaccctgagctctgggcccacaagccatggaagactggatcttgcttct

SEQ ID NO: 11347 - RNA, 7068 nt, Homo sapiens
  source 1..7068: mol_type = other RNA
ctgaatagctgggactacaggtgcccgccaccaggcccggctaattttttgtttgtttttttagtagagacggggtttcactatgttagccaggatggtctcgatctcctgatctcgtgatctgcccgcctcggcctcccaaagtgctgggattacaggtgtgagccaccgcacctggccccgagatttttaaataagttttgaacatgaataaaaatatggtgctcacatttattactttaaagaaagagactcgtctatcaaaaatttgatacaagtttttcacttattttcaaacatctactagaataattttcattcttccaggtgttcaaagtgcccaagcaggatgtaggttagttctacccttaaacttaaggtgtagattataagcacgttttccatttgcaacacaacagtaggcattcttgttaaattagtttgagaaatttgttttattttgtacaaggtacaatccctctgcacagtgaacatatattacaaatctgtgatttaaaaaagtattgccgtttcatagtctcattaatacctctgtacaataatggtttttctttcattcattttaattgtacacatattaattttttgaaaatttagtttctgaaaaataattgaacagatctttcaaagtcacccataaaatgcacagtatacatgtttaggctgaccatgaacctatttgtgatggtgttagacagaagtttctaacagttgctttgtaagattgaaatgtcttttactgataactgttcgataggggaaggcagctattgtcaccataatcacaccctctgcctttcccttctcctctgtattgcctggtttgacttgtattacatttccttaaaaagtcatggactgctagagctgaagggttagtagagctgtcttcccactctctgcttctcccctttttatgcataggaaaaaagggagcccagagagggcgactaacttgaccagagtaacactgaaatctcttgattcagtgtctagccattccacctcttgctgaatacctttgcccagaggatagttgacaaaagcggcgaaacttcaaacttgagtgatgctgcttgtttgcagtttgccaggcagcagttattgtacatgcaggataagggaagaagagaaaacctgggattgagttgaagtttctccttgctgatctgacatcttcatgctgctcatccttgcttcacaaacacttgctgccctgaaatactgaggtaagctgcttacctatatttctttctacatatgtatgagaaatatttacttgggtctccaaagtaattttctaatatttatattttaataaggcttttttggaaagtaaatttactattgctactcagttgctcccatgcacacatgcaacattcatgtaagtattacatattttcctctaacagtaaaatctgcttatgccttgagtgatgtgggaaggggagatgtactcatttatttatttttttgctttttctgattattgcccaaagtattgtgttccatggcaggcttccagtttctatcaagggtttcagaactctcatacttcctgtagcagtattccagcttcgcagtcatttagttcctcttctgtgtatctttttggaagtgttttttactggctggactgtaccagtgaatagagtggtacaggagtagccgttagcttcctaggtttgccctttttgtttttaattcttgtgagaaggttctctttagggcttgggagttgatttcatttcatttggacttatctgagcctcagtttatctgtgttcatagtggaaggtatagacacatctgaatactgggatctggagcattagctcattgtaatgcatattgggctagctcagtaagtagtagttttaagatagaaggtggaaggacttcatatcctcatgctgtttacagtaacgtttttacatcacgttacagcaactggttacagtccattctttttttgatcatttagttccattaaaaagcataatgtactttaagcagtgtaaacttgctgtatccacatttgtccaatttcctgtatacttttaggtttcatactacgtcaatctcaagatttatgaagaacttgaaagcaagtactcttgagtcaagggatgctgaccaaataaaatgaggaggccaactagccgtcttttacttaatcccgaccagtctatgactgcttgcttaaaggatcatcttagagctctgttttacatggaatgattcaggtgtcggatggactaagtagatatgacaaagccaggactaacttgtaatgtccttgaactttgaattggcaaaatttgataaagctgccctaggaatcttattgtagactgaaagagacactgctgcactttggaaacgtgtgtgtgtgtctctgtgtgtttaaacctatcacttagggggcagaagaaagtaaagtcttgttttttaaaatagaagttgtcagcattagactatatagattctgtaatcttggctgttgtaatttgatggaccagacagatatgtacagacattttaagactgttctgtttaagaacagttcatgtctgtgtactaattgtcttcggtaataaaacagatgttgatggtaacagcaaccaaaagtacatatacgtttcaggtgctttaaagtaatcctcttccctccccagtctcctttttgtcctaggaaggtttgttaaacctacatgtttttaaaatatcacgtttcagataaatatatatatatatatcagctatatttagctgatgttgatgagtagctgtatcttaaaatgttttaaaaatcatataatccagggcatttggggctgagtgggtgataggatttgcctttgagaacacaattccttgaacaattatcccagtcccacctggacgctcttctttagttccaggtgaacgtaataactaacatgcagctggagccagtctgtaccattacttcaagtcaagggactgtcttctttcagagtcagaatattcagtagagcacactgcaagagagaagcttatccctcttaagattgcttgtcctgggacggcccattggcagggctctgtcttactgggaggaggtcataatgaccaggaatatggctgttcctaggtaggtcgtatgcattctggatatagctggagttatgaccgcaaccttcttggaccacactgactgtgggctcaacttcatatatatttttattagatgtcgacaaggatggcacatctgtgtacggagaccccatgtgcacaggcgacttcatttctacatagctgctttctggaagcttgcaggtgaggatgggtgggtccttaattgtggcgtaagggttttcactgctattcaaggaacaagtactagaactgcacacggattctttcatgtaatctttgaagcctttgtccataatgtatgtgttctgacgtctatccattccacaagcacctggtgagtgtggctcagcggggcggctgaggtgtctaagttcaatgtagaagtcctcgggcgggtacctggcctccagggcactgatctggaaatgggagtctaacacgttcacatagctgtagggggtccagcctgctgtgtctctgtcaagggacttgttactgagcttggtggggctgttcctgtccagagtgctggcctggctggtggcaggccccccacatgccagtgcgtggtagctggaattggaaaagcagtgggcatggctgctactttgagacaaatctgagagggagtagtcggtgctggtcatcctcatggcaggtgtgtaggagacacggggagccaggtctcggcccttctctttctgccgccgccgatgccaggcaaataggcccagcagcaccacaatgaggaataacaggagcatgatgcctgtgacagcacccaccgagtgccgctctgcacccagtgctgggctgatcttggtgtagggattcagctcctccatcatgagggcagcttggtcacacctgattcctttgaagccagggctgcagtaacaggtgccggtgacatggtcacaggtggagttgttcatgcactcacatagctgctgacacccatagccaaaggttcctggggcacatctctgctcacagtgttgcccggtgaagcctgtgcggcaggtgcacttgccactgatgtggtcacagctggcgccattctgacactggcatacgcgcccacagtccttcccaaaaaatgctgctgggcagcgctgtgtgcagaagagtccagtccagccaggggtgcagtggcaggccccgtcctcggcgctgcagctcgccccgttgtggcagctgcatgcgtggaagcaggcggggccccagaacccgggtgggcaagcctgtgagcagtccttgccaatccatccaggaaagcactggcaggagccatcgatagggctgcaggtcccgttgttggcacaggagcagagctgggcacagtcctgcccaaagtatcctccagcacacacttggttgcagagagctccagagaatcctgggaggcactcacagatgccgctgatgtggtggcagggcctgctgctgtgcacgcagagggggcatggctgggcgcagccgtggccatagaacccaggggggcagattctctggcataagggtcctcggaagccaggggcacactcgcagctcccatcctctggggagcaggagcctccattctcacagctgcaggagacagagcagttggggccccagcggccaggtggacacgtgctgtcacagcggatgcctgggtggtggcacagcaagggaaggttacctgtccatccggccaggcagcagcagtggcctgtgacggggtcacatccatcagcatggctgcagtcacagtgttcactgcagttcagcccaaatgtgccatccgggcaaggcagctcacaggtgtctcccagccagccaggagtgcaggagcaggagccgtctatggggctgcaggctgccccattggcacaggtgcagctctcgttgcagttcaggccccacgtcccactgggacatggcagggtgcagtccaggccctgccacccttccttgcaggtacaggagccatctactggggagcaggtgccaccattgttacagctacagatggacgagcagttggggccataggtccctgctgcacaggaaacggcacagacctctcccatgaagcccggagcacaagtgcagcccccagtgatgctgtggcagtcggcgccattctgacaggtgcaaggcagctggcagccatcgccatagtagccaacagggcaggattcattgcagtggtgaccagaccagcctggctggcaggtacaagctccagttactgggtggcagctgatggtgttgtcagcgtcacaggggcagggcagggtgcagcctgggccatgcaggccctccgggcacagtcgctcctggcagcgtgggcccttgtagccaggctcacactcgcaggcacccgtggtgggtgaacactgccccccattgtggcagtcacagtgctgtgagcactggaagccgaaggacccgaaggggcactcctcttggcacctgtcccccatgtatccagctgtacagtggcactgtccagtcacgtggtcacactgccctccatggtggcaaggacaatcctggctgcagttctggccaaatgtccctggtgggcagggctgggcacacactgctccaaagaaaagaggaataggagacaaaggatgtcacacactggaagatggaaaagcaggtggaggagtgataactgctttggtttctgcttcctgggcaatgttaagtgcctgcaaagggagcgtcacaatgctggatgatgaaatcctttgtaacctcaaaaagctcaggaatcagagacactgggaccctccgaaggtgaaggtgcaggtatgatcaaaacaggactgtttgaaagtttataaaatagggaattagacccccaatctctgcccccaccttgaatagcagccaggtgaattgtccaagtctttcagagaggttggtgtcacaggctgtggacaagggacacaggcacagatgaaggtgggggtggaactctcctgctgctctcttccctgctgcgctcctaaaggctgactgccggactgaactccctgtggcaggaggttggagggttcctttctagggacactgaggagctcaagagaaatgacctaaagatattgatagttgagggtcccatcagtcaacacgcctgacatctccctccacccccaggtgtccaattggcttttctggggctcactgtaaaacatgaacagatggccaaggatcaccagatatttgaaataggccctcacatgaaagagaaacactgaaataaacaaataggcaacaggaacacagaggaaataggaaccatgcctggagcaaggaaaacctaaaaaaagagaaggaaaaaagcctctgtcataattaaaatgaacatgctcatgtagctataagaaaacattgcacctatgaaagaacagagtgctataaaataggatatccagagaataggaaagaggtcttgaaaattaaaaataaaatggtggaaattaaaatgttgcaatagaagagccaaaacataaagttgaggaaatttataaagtataccagagagagagagacaaagatagagagatgagattaaaaataatagagaaaatatagaggaccaattcaggtggtctgacatctaattaacaggagttccagacagtagaacagagaaaatagaggtgagtaaattgatggaaaatataataaaatttcccagaatggaaggatggagaacctgggtttctgaactgaaaaggcctacaaagtctttagcaaaaatataaaacaagacccacatcaaggcatgttatcgtaaacttttatatctctgtggataaagaaatgatgttaacagattttagaaagaggaaaacaggctaggtatggtggctcatgcctataattctagcactttgggag

SEQ ID NO: 11348 - RNA, 7030 nt, Homo sapiens
  source 1..7030: mol_type = other RNA
ctgaatagctgggactacaggtgcccgccaccaggcccggctaattttttgtttgtttttttagtagagacggggtttcactatgttagccaggatggtctcgatctcctgatctcgtgatctgcccgcctcggcctcccaaagtgctgggattacaggtgtgagccaccgcacctggccccgagatttttaaataagttttgaacatgaataaaaatatggtgctcacatttattactttaaagaaagagactcgtctatcaaaaatttgatacaagtttttcacttattttcaaacatctactagaataattttcattcttccaggtgttcaaagtgcccaagcaggatgtaggttagttctacccttaaacttaaggtgtagattataagcacgttttccatttgcaacacaacagtaggcattcttgttaaattagtttgagaaatttgttttattttgtacaaggtacaatccctctgcacagtgaacatatattacaaatctgtgatttaaaaaagtattgccgtttcatagtctcattaatacctctgtacaataatggtttttctttcattcattttaattgtacacatattaattttttgaaaatttagtttctgaaaaataattgaacagatctttcaaagtcacccataaaatgcacagtatacatgtttaggctgaccatgaacctatttgtgatggtgttagacagaagtttctaacagttgctttgtaagattgaaatgtcttttactgataactgttcgataggggaaggcagctattgtcaccataatcacaccctctgcctttcccttctcctctgtattgcctggtttgacttgtattacatttccttaaaaagtcatggactgctagagctgaagggttagtagagctgtcttcccactctctgcttctcccctttttatgcataggaaaaaagggagcccagagagggcgactaacttgaccagagtaacactgaaatctcttgattcagtgtctagccattccacctcttgctgaatacctttgcccagaggatagttgacaaaagcggcgaaacttcaaacttgagtgatgctgcttgtttgcagtttgccaggcagcagttattgtacatgcaggataagggaagaagagaaaacctgggattgagttgaagtttctccttgctgatctgacatcttcatgctgctcatccttgcttcacaaacacttgctgccctgaaatactgaggtaagctgcttacctatatttctttctacatatgtatgagaaatatttacttgggtctccaaagtaattttctaatatttatattttaataaggcttttttggaaagtaaatttactattgctactcagttgctcccatgcacacatgcaacattcatgtaagtattacatattttcctctaacagtaaaatctgcttatgccttgagtgatgtgggaaggggagatgtactcatttatttatttttttgctttttctgattattgcccaaagtattgtgttccatggcaggcttccagtttctatcaagggtttcagaactctcatacttcctgtagcagtattccagcttcgcagtcatttagttcctcttctgtgtatctttttggaagtgttttttactggctggactgtaccagtgaatagagtggtacaggagtagccgttagcttcctaggtttgccctttttgtttttaattcttgtgagaaggttctctttagggcttgggagttgatttcatttcatttggacttatctgagcctcagtttatctgtgttcatagtggaaggtatagacacatctgaatactgggatctggagcattagctcattgtaatgcatattgggctagctcagtaagtagtagttttaagatagaaggtggaaggacttcatatcctcatgctgtttacagtaacgtttttacatcacgttacagcaactggttacagtccattctttttttgatcatttagttccattaaaaagcataatgtactttaagcagtgtaaacttgctgtatccacatttgtccaatttcctgtatacttttaggtttcatactacgtcaatctcaagatttatgaagaacttgaaagcaagtactcttgagtcaagggatgctgaccaaataaaatgaggaggccaactagccgtcttttacttaatcccgaccagtctatgactgcttgcttaaaggatcatcttagagctctgttttacatggaatgattcaggtgtcggatggactaagtagatatgacaaagccaggactaacttgtaatgtccttgaactttgaattggcaaaatttgataaagctgccctaggaatcttattgtagactgaaagagacactgctgcactttggaaacgtgtgtgtgtgtctctgtgtgtttaaacctatcacttagggggcagaagaaagtaaagtcttgttttttaaaatagaagttgtcagcattagactatatagattctgtaatcttggctgttgtaatttgatggaccagacagatatgtacagacattttaagactgttctgtttaagaacagttcatgtctgtgtactaattgtcttcggtaataaaacagatgttgatggtaacagcaaccaaaagtacatatacgtttcaggtgctttaaagtaatcctcttccctccccagtctcctttttgtcctaggaaggtttgttaaacctacatgtttttaaaatatcacgtttcagataaatatatatatatatatcagctatatttagctgatgttgatgagtagctgtatcttaaaatgttttaaaaatcatataatccagggcatttggggctgagtgggtgataggatttgcctttgagaacacaattccttgaacaattatcccagtcccacctggacgctcttctttagttccaggtgaacgtaataactaacatgcagctggagccagtctgtaccattacttcaagtcaagggactgtcttctttcagagtcagaatattcagtagagcacactgcaagagagaagcttatccctcttaagattgcttgtcctgggacggcccattggcagggctctgtcttactgggaggaggtcataatgaccaggaatatggctgttcctaggtaggtcgtatgcattctggatatagctggagttatgaccgcaaccttcttggaccacactgactgtgggctcaacttcatatatatttttattagatgtcgacaaggatggcacatctgtgtacggagaccccatgtgcacaggcgacttcatttctacatagctgctttctggaagcttgcaggtgaggatgggtgggtccttaattgtggcgtaagggttttcactgctattcaaggaacaagtactagaactgcacacggattctttcatgtaatctttgaagcctttgtccataatgtatgtgttctgacgtctatccattccacaagcacctggtgagtgtggctcagcggggcggctgaggtgtctaagttcaatgtagaagtcctcgggcgggtacctggcctccagggcactgatctggaaatgggagtctaacacgttcacatagctgtagggggtccagcctgctgtgtctctgtcaagggacttgttactgagcttggtggggctgttcctgtccagagtgctggcctggctggtggcaggccccccacatgccagtgcgtggtagctggaattggaaaagcagtgggcatggctgctactttgagacaaatctgagagggagtagtcggtgctggtcatcctcatggcaggtgtgtaggagacacggggagccaggtctcggcccttctctttctgccgccgccgatgccaggcaaataggcccagcagcaccacaatgaggaataacaggagcatgatgcctgtgacagcacccaccgagtgccgctctgcacccagtgctgggctgatcttggtgtagggattcagctcctccatcatgagggcagcttggtcacacctgattcctttgaagccagggctgcagtaacaggtgccggtgacatggtcacaggtggagttgttcatgcactcacatagctgctgacacccatagccaaaggttcctggggcacatctctgctcacagtgttgcccggtgaagcctgtgcggcaggtgcacttgccactgatgtggtcacagctggcgccattctgacactggcatacgcgcccacagtccttcccaaaaaatgctgctgggcagcgctgtgtgcagaagagtccagtccagccaggggtgcagtggcaggccccgtcctcggcgctgcagctcgccccgttgtggcagctgcatgcgtggaagcaggcggggccccagaacccgggtgggcaagcctgtgagcagtccttgccaatccatccaggaaagcactggcaggagccatcgatagggctgcaggtcccgttgttggcacaggagcagagctgggcacagtcctgcccaaagtatcctccagcacacacttggttgcagagagctccagagaatcctgggaggcactcacagatgccgctgatgtggtggcagggcctgctgctgtgcacgcagagggggcatggctgggcgcagccgtggccatagaacccaggggggcagattctctggcataagggtcctcggaagccaggggcacactcgcagctcccatcctctggggagcaggagcctccattctcacagctgcaggagacagagcagttggggccccagcggccaggtggacacgtgctgtcacagcggatgcctgggtggtggcacagcaagggaaggttacctgtccatccggccaggcagcagcagtggcctgtgacggggtcacatccatcagcatggctgcagtcacagtgttcactgcagttcagcccaaatgtgccatccgggcaaggcagctcacaggtgtctcccagccagccaggagtgcaggagcaggagccgtctatggggctgcaggctgccccattggcacaggtgcagctctcgttgcagttcaggccccacgtcccactgggacatggcagggtgcagtccaggccctgccacccttccttgcaggtacaggagccatctactggggagcaggtgccaccattgttacagctacagatggacgagcagttggggccataggtccctgctgcacaggaaacggcacagacctctcccatgaagcccggagcacaagtgcagcccccagtgatgctgtggcagtcggcgccattctgacaggtgcaaggcagctggcagccatcgccatagtagccaacagggcaggattcattgcagtggtgaccagaccagcctggctggcaggtacaagctccagttactgggtggcagctgatggtgttgtcagcgtcacaggggcagggcagggtgcagcctgggccatgcaggccctccgggcacagtcgctcctggcagcgtgggcccttgtagccaggctcacactcgcaggcacccgtggtgggtgaacactgccccccattgtggcagtcacagtgctgtgagcactggaagccgaaggacccgaaggggcactcctcttggcacctgtcccccatgtatccagctgtacagtggcactgtccagtcacgtggtcacactgccctccatggtggcaaggacaatcctggctgcagttctggccaaatgtccctggtgggcagggctgggcacacactgctcctggaagatggaaaagcaggtggaggagtgataactgctttggtttctgcttcctgggcaatgttaagtgcctgcaaagggagcgtcacaatgctggatgatgaaatcctttgtaacctcaaaaagctcaggaatcagagacactgggaccctccgaaggtgaaggtgcaggtatgatcaaaacaggactgtttgaaagtttataaaatagggaattagacccccaatctctgcccccaccttgaatagcagccaggtgaattgtccaagtctttcagagaggttggtgtcacaggctgtggacaagggacacaggcacagatgaaggtgggggtggaactctcctgctgctctcttccctgctgcgctcctaaaggctgactgccggactgaactccctgtggcaggaggttggagggttcctttctagggacactgaggagctcaagagaaatgacctaaagatattgatagttgagggtcccatcagtcaacacgcctgacatctccctccacccccaggtgtccaattggcttttctggggctcactgtaaaacatgaacagatggccaaggatcaccagatatttgaaataggccctcacatgaaagagaaacactgaaataaacaaataggcaacaggaacacagaggaaataggaaccatgcctggagcaaggaaaacctaaaaaaagagaaggaaaaaagcctctgtcataattaaaatgaacatgctcatgtagctataagaaaacattgcacctatgaaagaacagagtgctataaaataggatatccagagaataggaaagaggtcttgaaaattaaaaataaaatggtggaaattaaaatgttgcaatagaagagccaaaacataaagttgaggaaatttataaagtataccagagagagagagacaaagatagagagatgagattaaaaataatagagaaaatatagaggaccaattcaggtggtctgacatctaattaacaggagttccagacagtagaacagagaaaatagaggtgagtaaattgatggaaaatataataaaatttcccagaatggaaggatggagaacctgggtttctgaactgaaaaggcctacaaagtctttagcaaaaatataaaacaagacccacatcaaggcatgttatcgtaaacttttatatctctgtggataaagaaatgatgttaacagattttagaaagaggaaaacaggctaggtatggtggctcatgcctataattctagcactttgggag

SEQ ID NO: 11349 - RNA, 7679 nt, Homo sapiens
  source 1..7679: mol_type = other RNA
ctgaatagctgggactacaggtgcccgccaccaggcccggctaattttttgtttgtttttttagtagagacggggtttcactatgttagccaggatggtctcgatctcctgatctcgtgatctgcccgcctcggcctcccaaagtgctgggattacaggtgtgagccaccgcacctggccccgagatttttaaataagttttgaacatgaataaaaatatggtgctcacatttattactttaaagaaagagactcgtctatcaaaaatttgatacaagtttttcacttattttcaaacatctactagaataattttcattcttccaggtgttcaaagtgcccaagcaggatgtaggttagttctacccttaaacttaaggtgtagattataagcacgttttccatttgcaacacaacagtaggcattcttgttaaattagtttgagaaatttgttttattttgtacaaggtacaatccctctgcacagtgaacatatattacaaatctgtgatttaaaaaagtattgccgtttcatagtctcattaatacctctgtacaataatggtttttctttcattcattttaattgtacacatattaattttttgaaaatttagtttctgaaaaataattgaacagatctttcaaagtcacccataaaatgcacagtatacatgtttaggctgaccatgaacctatttgtgatggtgttagacagaagtttctaacagttgctttgtaagattgaaatgtcttttactgataactgttcgataggggaaggcagctattgtcaccataatcacaccctctgcctttcccttctcctctgtattgcctggtttgacttgtattacatttccttaaaaagtcatggactgctagagctgaagggttagtagagctgtcttcccactctctgcttctcccctttttatgcataggaaaaaagggagcccagagagggcgactaacttgaccagagtaacactgaaatctcttgattcagtgtctagccattccacctcttgctgaatacctttgcccagaggatagttgacaaaagcggcgaaacttcaaacttgagtgatgctgcttgtttgcagtttgccaggcagcagttattgtacatgcaggataagggaagaagagaaaacctgggattgagttgaagtttctccttgctgatctgacatcttcatgctgctcatccttgcttcacaaacacttgctgccctgaaatactgaggtaagctgcttacctatatttctttctacatatgtatgagaaatatttacttgggtctccaaagtaattttctaatatttatattttaataaggcttttttggaaagtaaatttactattgctactcagttgctcccatgcacacatgcaacattcatgtaagtattacatattttcctctaacagtaaaatctgcttatgccttgagtgatgtgggaaggggagatgtactcatttatttatttttttgctttttctgattattgcccaaagtattgtgttccatggcaggcttccagtttctatcaagggtttcagaactctcatacttcctgtagcagtattccagcttcgcagtcatttagttcctcttctgtgtatctttttggaagtgttttttactggctggactgtaccagtgaatagagtggtacaggagtagccgttagcttcctaggtttgccctttttgtttttaattcttgtgagaaggttctctttagggcttgggagttgatttcatttcatttggacttatctgagcctcagtttatctgtgttcatagtggaaggtatagacacatctgaatactgggatctggagcattagctcattgtaatgcatattgggctagctcagtaagtagtagttttaagatagaaggtggaaggacttcatatcctcatgctgtttacagtaacgtttttacatcacgttacagcaactggttacagtccattctttttttgatcatttagttccattaaaaagcataatgtactttaagcagtgtaaacttgctgtatccacatttgtccaatttcctgtatacttttaggtttcatactacgtcaatctcaagatttatgaagaacttgaaagcaagtactcttgagtcaagggatgctgaccaaataaaatgaggaggccaactagccgtcttttacttaatcccgaccagtctatgactgcttgcttaaaggatcatcttagagctctgttttacatggaatgattcaggtgtcggatggactaagtagatatgacaaagccaggactaacttgtaatgtccttgaactttgaattggcaaaatttgataaagctgccctaggaatcttattgtagactgaaagagacactgctgcactttggaaacgtgtgtgtgtgtctctgtgtgtttaaacctatcacttagggggcagaagaaagtaaagtcttgttttttaaaatagaagttgtcagcattagactatatagattctgtaatcttggctgttgtaatttgatggaccagacagatatgtacagacattttaagactgttctgtttaagaacagttcatgtctgtgtactaattgtcttcggtaataaaacagatgttgatggtaacagcaaccaaaagtacatatacgtttcaggtgctttaaagtaatcctcttccctccccagtctcctttttgtcctaggaaggtttgttaaacctacatgtttttaaaatatcacgtttcagataaatatatatatatatatcagctatatttagctgatgttgatgagtagctgtatcttaaaatgttttaaaaatcatataatccagggcatttggggctgagtgggtgataggatttgcctttgagaacacaattccttgaacaattatcccagtcccacctggacgctcttctttagttccaggtgaacgtaataactaacatgcagctggagccagtctgtaccattacttcaagtcaagggactgtcttctttcagagtcagaatattcagtagagcacactgcaagagagaagcttatccctcttaagattgcttgtcctgggacggcccattggcagggctctgtcttactgggaggaggtcataatgaccaggaatatggctgttcctaggtaggtcgtatgcattctggatatagctggagttatgaccgcaaccttcttggaccacactgactgtgggctctaagaaatatagtgaaaaatgagttcagagaacagattagctttggttgccttgttggagaggaagagagttctacttaacttggggaaaggagccagggatttataaatctatggcaaatacatgagggttaggactgaggcttgctcaggagatggaaaactaagtgaatgtgctgtcaacatccaagcctctcatcaacaccaaaggatttaaaatatcctagaggtaggagtcttaccagtgagcccagggacataaactgggagaaggtagaaggtgatttagagacttgttgatgtctctgattgctttcttttttaaaatgagatttgtatcaacaatctgtgtgtgtgtgtgcgcgcgtgcacgtgcatgtgcccatttcccacccccagtatttgtttcatattagtcctggtgttttttaaagcagagttggtacaataatttgacttcctgcattagctaggagggtagtcctaggaaagacagttcaccttagagatgcctttaaaagcaacaaaagaaggatgtgtggtcaaggtggggtgagtggagagggcttgcttttacttcaaatgctgcactattgccctgatttcactaagttacttatttgagacacctaccaacttcatatatatttttattagatgtcgacaaggatggcacatctgtgtacggagaccccatgtgcacaggcgacttcatttctacatagctgctttctggaagcttgcaggtgaggatgggtgggtccttaattgtggcgtaagggttttcactgctattcaaggaacaagtactagaactgcacacggattctttcatgtaatctttgaagcctttgtccataatgtatgtgttctgacgtctatccattccacaagcacctggtgagtgtggctcagcggggcggctgaggtgtctaagttcaatgtagaagtcctcgggcgggtacctggcctccagggcactgatctggaaatgggagtctaacacgttcacatagctgtagggggtccagcctgctgtgtctctgtcaagggacttgttactgagcttggtggggctgttcctgtccagagtgctggcctggctggtggcaggccccccacatgccagtgcgtggtagctggaattggaaaagcagtgggcatggctgctactttgagacaaatctgagagggagtagtcggtgctggtcatcctcatggcaggtgtgtaggagacacggggagccaggtctcggcccttctctttctgccgccgccgatgccaggcaaataggcccagcagcaccacaatgaggaataacaggagcatgatgcctgtgacagcacccaccgagtgccgctctgcacccagtgctgggctgatcttggtgtagggattcagctcctccatcatgagggcagcttggtcacacctgattcctttgaagccagggctgcagtaacaggtgccggtgacatggtcacaggtggagttgttcatgcactcacatagctgctgacacccatagccaaaggttcctggggcacatctctgctcacagtgttgcccggtgaagcctgtgcggcaggtgcacttgccactgatgtggtcacagctggcgccattctgacactggcatacgcgcccacagtccttcccaaaaaatgctgctgggcagcgctgtgtgcagaagagtccagtccagccaggggtgcagtggcaggccccgtcctcggcgctgcagctcgccccgttgtggcagctgcatgcgtggaagcaggcggggccccagaacccgggtgggcaagcctgtgagcagtccttgccaatccatccaggaaagcactggcaggagccatcgatagggctgcaggtcccgttgttggcacaggagcagagctgggcacagtcctgcccaaagtatcctccagcacacacttggttgcagagagctccagagaatcctgggaggcactcacagatgccgctgatgtggtggcagggcctgctgctgtgcacgcagagggggcatggctgggcgcagccgtggccatagaacccaggggggcagattctctggcataagggtcctcggaagccaggggcacactcgcagctcccatcctctggggagcaggagcctccattctcacagctgcaggagacagagcagttggggccccagcggccaggtggacacgtgctgtcacagcggatgcctgtccatccggccaggcagcagcagtggcctgtgacggggtcacatccatcagcatggctgcagtcacagtgttcactgcagttcagcccaaatgtgccatccgggcaaggcagctcacaggtgtctcccagccagccaggagtgcaggagcaggagccgtctatggggctgcaggctgccccattggcacaggtgcagctctcgttgcagttcaggccccacgtcccactgggacatggcagggtgcagtccaggccctgccacccttccttgcaggtacaggagccatctactggggagcaggtgccaccattgttacagctacagatggacgagcagttggggccataggtccctgctgcacaggaaacggcacagacctctcccatgaagcccggagcacaagtgcagcccccagtgatgctgtggcagtcggcgccattctgacaggtgcaaggcagctggcagccatcgccatagtagccaacagggcaggattcattgcagtggtgaccagaccagcctggctggcaggtacaagctccagttactgggtggcagctgatggtgttgtcagcgtcacaggggcagggcagggtgcagcctgggccatgcaggccctccgggcacagtcgctcctggcagcgtgggcccttgtagccaggctcacactcgcaggcacccgtggtgggtgaacactgccccccattgtggcagtcacagtgctgtgagcactggaagccgaaggacccgaaggggcactcctcttggcacctgtcccccatgtatccagctgtacagtggcactgtccagtcacgtggtcacactgccctccatggtggcaaggacaatcctggctgcagttctggccaaatgtccctggtgggcagggctgggcacacactgctcccgtccagcctggggggcaggcacactcgccagtgatgtggtggcaggtgcccccattctgacaggggcagcgcagctcacagtgagctccatggctcccaggagggcacagctcctcgcagtagacgccggtgtagccaggtgcgcagaggcactcgccggcgcgggggtcgcagctggcaccgtgtcggcactggcacggcagctggcatcccttgccgtgggtgccaggtgcgcagagctcctcgcagcgccatccacggaagccggcggcgcacacgcaggcgcctgtgatggggttacacagggcgccgttctggcactggcaccggttgctgcagtggggcccccagtggtcgctgtcgcagccgctggagcagtcgggccctccccagccaggctcgcagtggcaggtgtccggggaaacgcagcggccgtgcacacactcctccgtacacaggggtatgcagaagtctccgctctcatagtagccagggcagcactgggacctccgccggtacatggtccggaggcctctccgatacgccgtcttataactgatccggtgcctggtgcacttgaaccagttgaggatgtctgtgcatcgtgtgtaatagatctgatcgaaggggtgtgcatacgattcctggacagtcacagcatagctctcccagtggctgcacacgttggggtcctcggggttcagggcaagggtggcttgcaggaaggagaaggcaatgagccccgtcagggagagcaccatcccgggccctgcacaggagaacaaaggaggctgcgtctgtgatcagaccatgttcctggcaactacttagtttcccatcgtcgtgggtaatgagcatttgatatttcacattgcaggctttgactaacactgtaacagttcactggttctgagtaacaggagagtgggaagcctgagtcaggaaaaagtccaaattctaggccaggggttctgaatgttttttgactcagggactgctctgagaatccagtgaaaggtatagatgttctctccaggaaaatgcccacaagtgcaaaatcggctataattgcagggtgtcctcaggcccccgggcccatccttggacccagggaccccagatctggactgctttaaagggaatgccctccccattcccttatccctcatcattgacattctttgcccatctacttcctttccctactccctcctgccaaggagaaagagaaaaaagatgtctggtgtggacctggggggaaatgagccaagaaaaccctgagctctgggcccacaagccatggaagactggat

SEQ ID NO: 11350 - RNA, 10080 nt, Homo sapiens
  source 1..10080: mol_type = other RNA
ctgaatagctgggactacaggtgcccgccaccatgcccaactaatttttttgtttttagtagagacagggtctcaccatgttagccaggacggtcttgatctcctgacctcgtgatccgcccgcctcggcctcccaaagtgttgggattacaggcgtgagccactgcgcctggctaatttttgtatttttagtacagaaggggatttgccatgttcatcaggctggtctcgaactcctgacctcaggtgatctgcccaccttggcctcccaaagtgctgggattacaggcgtgagccactgcgtctggcctcaatctctacattatatcagatgacaattaaggaatttttccagaaacattttctgtatagccagaaaaaaattaaaaataacaagccacattgatctctaataatatttcaaatgaagacattcacttgcccatggcaatctggcaactatatttatgtaataaacctaagaatgcagtttaagaataattactgaacaaaaaattttcaatcaactcctctgaaatttcttttacattttataattattttaatattggtaaattgaattgcttttaaattagccatacgaaccattgctttgttcactaatttgatcttgaatacattttgtgtaaattttaggctaactagctatattcatatttaagagaacaaagaccacaaaacgttatgtcattcttttctatgtatcaatttaaggtgcttatattggtgcttaagaagactttcccatttaaaaaagccatgtccaatatttataactttctttcatttttattatctgtaatataattttccttctttaaaattacttaaaatcactaatggaaaaacagttgataaaatatctgaatcccatcaatttacatgtaaatgacgttaataatacaggttgatctagtaaaataatacaagttgatctagttcatgggatgaataagaagaataaaaatgagaccaaaataatgattataaaatggtcaaatgagaaccaaatgagagctgggcggaattttagacgctacctaaactaattctcttgttccctagagaatgagaaaaatggaggcaccacgagataaaatgccttatccaaagttacacagctaactgcaaaagagaggcaagagtagaagtcaagtttcctgactcaaaatcctattgtatttttaaaaataaaataatacagttttactaatcattaaaaaaatcctgccaatttagaaaatagatttttttgtttaattttagactccaggatagaaaatagaaattattaagctctaagttaaaaaaaaaaaccaataagcacaacacaaagaaatatctgcaatttagcatatacaaacaagctgacttatacaacaaaaaaccttaaagctacaataataataaagtaatccatcctactccaggaatatgataaaatatcaaccttaaaaaaactttaaaaactaactttactagttaatggtaattagcaaaataatgaaacagtgaatcttcaaaatctgaattatttcaaggtaaaaaacatttttaatctttatcgggaaaaactggtgacagtgaccaataaaatgagcataaagtataagcaacgctttcacaccaacaaaaaaattcaagaaagaatttcctgaggcagatgatgatttaaaaagtaatctgaaggaaattatccttcaatgcctttcaacagattgaactactgtgtcttataggaagtaagtaatgcagtggtttggtgtttgactaaaatataagtgaaaactttcttttatatttatggcaacagaattttactttctaattagagatcacagaataagaaacatgtttaactcatattaaatctttatatattaaatctttataaatcaaccaaatagaaatgtctacaaggatggctggttctgggtagacttcaacattttcattcttagaagacttggatcctgagagaaaattgtaatcctatatcaatttgatgactaaagaagcacaggattaagattaaattagtaaaaaacccaggagactgattacaatcagacggaaggcatgcgatacctagtcttcctactcctttcccaaattcatctaatcggaacaaaagaaggagagaagagaattaaattatgaagagatgccaatacaattattttcatataaaataggtcaaaattatataagaataatgtgtaagattatacagctactaggaaatacagctgaattaaatgtaaacattttttcttaatcagctgtaaaacgacacaaaagcattgaaaagaatcacaagttcctttgtaaatctaggttccataaaaatgctatcctttgtgagtgaagaatggagaaaaaatccttactttacatactttaaaaaaattataaatgtgtacaaacaattctcatagtgtgatgacttaaaatttaaagttttgccacaatgaaaaccaacaagtgaatcactttttcaaaactttttctcaatcagaaaaaatgaggtacataaaagccaaaaagtcaaagacaaaaaacattatagggtctacattcttcttcatatatatttttttttataatttaagtcaagctaatgtacttatacaatttcatataaaaggaaaaataaaatgaatatccccaaatttgttctacaaattcaactacataaaatttgaggcatactctggtataacacatattaaagaaccaatacaatttaagagcataacctactttttaaaggttaattggatgaccgatttaaagactgtaccaaatgaacactggtctaattgcctattttgttgttattgctaaaaagaaatactaatgaagactgtaaccttgttttctatagcccccccaaattctaacaaaaccaaatggtatcagtagaacaatttatggatcaggcatggtggctcatgcttgtaatcccagtgctttaggaggccaggagttcaagaccagcctggtcaacatagtgagactcatctctacaaaaaattaaaaaaattaaaattaagccaggtgcagtgactcatgcctgtaatcctagcactttgggaggctgaggtgggcagatcacttgaggtcaggagtttgagaccaacatggcaaaactccatctccactaaaaatacaaaaactagctggatgtggtggcacgcacctgtagtcccagttactcgggaggctgagacagaagaatcacttgaacctgggaggtggaggttgcagtgagctgagattgtgccactgcactccagcctgggcaacaaagccagactccgtctcaaaaaaagaaaaaaaaattaaaattagccaggtgtagtggtgcatgcctacagtcttagctacttgggaggctgaagctggaggactgcttgagcctaggagttcaaggttataatgaactatgattatgccactgctctccagcctgtgtgacagagcaagaccctgtctctataaaaaatttttttaagtagaataatttatgggttacagagcattataataaatactatttcatttgatccttacaatatccagtgagggaggctaaaaccaaaaattaccttatccacattttacattgaagaaacaaagactcagagaaataaaatgaccagcccagttgacatcatgagtcttaaaattccaatcccaggggaattttcattacaccagactatgtaagtcatccaaatatggtaatatgtaaatgtacctttggcatgtcaaaaagcaatataaatatcatcataatgaaattttggtatgttaatattttctaagctccagcaaatgattcactaatttatataaaaaaaattaagtggttcctttcatttcacagagatatagcctaactaagatgggtacagtttgagttattttcagctattatcacaaagaaactgatgaggtaggttaaaatgtagtaaatttttctaatttgaagacattcttaggatttttataaatctgctctaagagcagcagaaaaagaaaggttgatttgaagattcatttactcagctggtccacaaagatctaacagcataagactaaaaggagtctaattactcacttctaagaatcactgttcatcttctaaaattaattaaaaggattggtacatgtctgtacatatatttctttaattataatagtgatatggactgttatctatgcaaaatatgtttcatttggtgtactttacatatttattacctgccacatattattctggtaaagcagagacttcatttcacataggttatagatctttcaaatttctttgatgtgagactcagtactagggtaaaagcaagttgtgtgacatgaattgttcatttaaatatttattgaaaaactgtgtatgaatccctgtgccagctgagttattaaccaattgttctttgaaacaaactgttttgagtttaatattatcttagatcttttgtctagttattgaataaaaaaagttgctgaaatcaaagtactttttgaaaaccttttgataatatattaacatgttagagagaactattattttctcagttgtcaactgaaaaaagaaaacactaaacattatcatatgccaatcaaagttaaacatatggtaggaaaactgtccagacttattcagattggtttaagctagttagacttaaaactgctgcccaaactgaatactgttgtttaaaaccatggattaatattacataaattttgtgggacaaaattaagatacttactgaaagtaactgaaaagtcaatatagtattcccatacatacccacaatttaatagagaaaatacaaatgattatctaaaaatctagaagcacaaagttaagattttcatagtgatgttcacttaactgtctatacttggcccacttgtaaaagaaaaccaattaacattttggcagttgataatataatgcagatggcaatggatgacaacatcttcgagcccaaactggtaccttctattttaacttatttttgtttgtgaatgtttgttttagttctctcatgctgtttgcaggagagattctcagacaaaagcttcatgaattattgataaataagttgttatatgtttggctttcagagaaaatgtttactaattgtcggttatgagggaattcagacctgcctgctttgagcattaactccagctccaaggagaaaggcaatgaacacagagaaaaatgaaaaacattttgggccaaatattcaaatatctctcatgaagaataagtcatattatcatacatgtactttgaaatatataacataatagacaaattattactatcagaaaactgactttgctgcctgatgagaatattctttttcaacacctaatttcttggcagtttgttttaaagggtaagaaagaaagtatacatgaattcaacacacgtcaaggaatgtactatagcagtcctcacacctcttaaatccacaataacctaatcccttatcattcataatgctttacagttttcaaagagctttcacataatttttttcacttgatcttaatctgacagctttgtgaggtaggtagagtacgtatttatcttctatcttcatttacaaacaagggaactgaggctcggagagttaaattgttaaaggtcataaactataatagcataaggcagagccaggcctcttcagagtctagaataattcttcaaagtatgattcttggattacctccgtaagaatcacctgcggtatttttataactacagattttaaagtcctatcactttggccttactgagtaagtctctctaggagtacagcccagaatttggcatcaggtgcagaacaactgaatattagataatgatataaaagcgaaagacagaatccatgtggatgttcatgtgatatatgatgccgacagatcatcaggggcaagttaaagtagtgagtttcaagccaggctgcagattagaatcacctggagcgctttttttttttttttttttttttaagaaagctaccaattcttatttgtatgagaggaaggtgttaggcatctgaagtaacccaagtgattcttatctgcagtcagggttgaggacccttgtttaaatatgctttttacataatacatcaagcatgttccagcatttttctttctcttctgattgatttcatgcctaataagttttacagtttatattgtaaattatttaaacattatcagataaacatttttacttgattttttaaagattaaatgatattcatactaagactaatcatgcttcatttagctacaacaattttcaaatactcaaatcaatcaccactttggactgaggttatatatatttcagttgtaaacaagaatgatccagaatctgaaaataagggtgtggggcaaaagctgtagcctactggctattgggcaaggcaagtgcagacaatcaactcactacaggagggcctggaagccaaggtctggtggctttggcaagatcacatctcactgtagaaaaatacaacaatgaatacagagaaaatgttttgccattttgtaattgtggttaccttataatgtatgatgtttatcttattacatgcctccacaaagcaaattttgaacattaagttctctatgaatcaatactattacatgggaaaagatggctacaaattaaaatttttccatcatgcatatggataagttataaaaacacagccagaaaaagtaatatttacaaaagttataaaaacagcacaattataggggaaacaatgcccatctctttattccactgctaatccaaaccctgaatatctctgcatgaagattatttcgatagaattttaagagaacctttcatagactaatcaaattcttctgttgcacttttattctattagctaaaatacccttgctgatttattaaattctcctacagtttaaaaacacagttcttttttcacttagtggaaataaaactacaaagtcctactgttcatctgagaagtaaaccttgcatagaaaatttctttaattctgaaattgttttattaactgagctaccagaatgttatctcacaactagtttatagtatatgaaagttcactacaaagcagtcaccacacatttaggatttttctaaatataaaatgagtgggtttataaaaatgcttaccagacaaataattatctcttcataacctagaaagacgaattatttttgtgatgatagaattcttagtgttttggatgccttgatgttccaagtttgatgcaatataaaaaagcaatcatttacctttccagtggacacaatctgtacttgactgaaagcatgttaactgtgagttacagctatcagtcatgcaaaaggcaaagaataaaatctgctttttaaacagcacaagatttccaccttagacaagacaaattaagcactggttccatcttcttcaataacccgattcatgctggtgccatgtgtgatatgagtcatgggattattactgagatctctgatgctgctatgtcgtgactgttcattgagccgatgagaactactatgcctggagtgatctgttagtcgtgacatgctgccatgaggtagtctctcctccattcctctgtaactgcagggcgtgtacctgccatcacgtgatctgtggaggctgccgtggtagctgctcactttgctgtggatgcttcctgctttgcttctttgatcatccaccatagccagctgagttgaagaagcatgggtggatgttccttgagtggaagttccccttgactttcttatgataggagtatttggatccctcaggagagactgagcaaaatcaggttcctggagtacctgtcggctctcattcactatctcttttttcctacgaccatgaaaaaaactggcccattcaaagcatgtctttttgcttccaacccaaaatacagagggaatgccaactatgagagccatcaggtatttcatcagaaagagaatcaagtctggacgactcatttgagtaacccatttccctcatggtcctttcataaacaattctgattccttttggaactgcctgatatggacatggaatgtgatattctctgcagcgttcttgtatccacgttgtttcccagatgccccggtaagcttgctcataaaagtagcatccaattacaaccaagagtggtacgagataaagaatgctgaaaacaccgatccggatcataaacttcactaatttatcttggttctccttttctaatggaatctcaattcgaactctgtttagggatataatgccagctaagaggagagaaaccccaactaccacatacaggcagaggggagcaagaacaaaatatctcaatgcatcaacatcgtagaggccaacaaaacacacgccactaatattgtcaccttcaattttattcatcgctaaaaggatgatggttagagttccggggatgccccatgcactggcgtgaaacagcaatgctttcttctcaatagcttcactaccccactttggcacagctgctaaaaaccatgtgatggtaagaattacccaccatacactgccagccatagtaaaaaaatagagtatcataaaaagcatggtacaggctttattatgagatccttgtgtcactgtggaagccttatattgtgcagggatggatgcattgcaggctactcgatcttcaagcaaaaatccaatgaagaaaattaaggataccatcatgtagcagactgcataaaatataataggcctttcaggataacggaatcttgtgacatcaatcaaaaaagttaaaaaagtaaacaatgtggccgagaggcaaatgattgaaatcaatcctatgaaatagcgagcaaatgacagttcttctcttctgaagtacatatttggacaaggaggtgaacaatcacgcacatgcagaaaagaataacccagatcaggatcaatttttaactctcggggacaccaaaaaccatagtctctctgcactgccactggggctccttcagttggttctccagctaaattcagatccacaagtcgaggatatggctcatcacaatctgggaacctactgcattccatatcttcaggccaaggaacaccaaacatctccatgagcttcgaacactcactgtaagcccgctgacacagcctacgacagggaagtgtgacacgtccatattccatacaaataggagcgtagagtgcacaaagaaaaggccggaaatcccgagaacaatccagattcaccatagggtggaatggctccattgccaaagctgctgtctgttggtcataatgattcagaagattaggcatgaaggtagtattataaggcaaatcttggcacatcctcaaggtaataggttcacaagaaaacaaactgtgcccacctatatgccccatgaacacagtcaagggccaaagagagaagacaatccaagtcatagccatccttcctgggtctgaaggagattcagatgatcaggcctattcaatatgtattttagatatttatacacctgcaggtctcagctcgaaggtacttcttctgtatcttactgttaaattcttcaaacagttaaatactcttcgcaccgtcagaggtttgttagcttggtctcacaaaaggcgtttgtttttggtttcacaatatgggaaaatgacatcatcttgtctcttcttttcattttattacatggggcacatttggccaacatatcaagttgatcaaccacattcccaaaccacagattccatcttaggagaagagctatttcttccttcaactgaaatatctcaggttacaagtgctccataagtcaggtcttgagaaatgctatcctcagaccccggcgcctggctccaaggggtgggggggctgcaccgcctgccgcgggcggccgcgcgtccctcaggtacccggagcggccgaggaacgccggcgcgcgcctcccagcgacagcgagcttt

SEQ ID NO: 11351 - RNA, 9985 nt, Homo sapiens
  source 1..9985: mol_type = other RNA
ctgaatagctgggactacaggtgcccgccaccatgcccaactaatttttttgtttttagtagagacagggtctcaccatgttagccaggacggtcttgatctcctgacctcgtgatccgcccgcctcggcctcccaaagtgttgggattacaggcgtgagccactgcgcctggctaatttttgtatttttagtacagaaggggatttgccatgttcatcaggctggtctcgaactcctgacctcaggtgatctgcccaccttggcctcccaaagtgctgggattacaggcgtgagccactgcgtctggcctcaatctctacattatatcagatgacaattaaggaatttttccagaaacattttctgtatagccagaaaaaaattaaaaataacaagccacattgatctctaataatatttcaaatgaagacattcacttgcccatggcaatctggcaactatatttatgtaataaacctaagaatgcagtttaagaataattactgaacaaaaaattttcaatcaactcctctgaaatttcttttacattttataattattttaatattggtaaattgaattgcttttaaattagccatacgaaccattgctttgttcactaatttgatcttgaatacattttgtgtaaattttaggctaactagctatattcatatttaagagaacaaagaccacaaaacgttatgtcattcttttctatgtatcaatttaaggtgcttatattggtgcttaagaagactttcccatttaaaaaagccatgtccaatatttataactttctttcatttttattatctgtaatataattttccttctttaaaattacttaaaatcactaatggaaaaacagttgataaaatatctgaatcccatcaatttacatgtaaatgacgttaataatacaggttgatctagtaaaataatacaagttgatctagttcatgggatgaataagaagaataaaaatgagaccaaaataatgattataaaatggtcaaatgagaaccaaatgagagctgggcggaattttagacgctacctaaactaattctcttgttccctagagaatgagaaaaatggaggcaccacgagataaaatgccttatccaaagttacacagctaactgcaaaagagaggcaagagtagaagtcaagtttcctgactcaaaatcctattgtatttttaaaaataaaataatacagttttactaatcattaaaaaaatcctgccaatttagaaaatagatttttttgtttaattttagactccaggatagaaaatagaaattattaagctctaagttaaaaaaaaaaaccaataagcacaacacaaagaaatatctgcaatttagcatatacaaacaagctgacttatacaacaaaaaaccttaaagctacaataataataaagtaatccatcctactccaggaatatgataaaatatcaaccttaaaaaaactttaaaaactaactttactagttaatggtaattagcaaaataatgaaacagtgaatcttcaaaatctgaattatttcaaggtaaaaaacatttttaatctttatcgggaaaaactggtgacagtgaccaataaaatgagcataaagtataagcaacgctttcacaccaacaaaaaaattcaagaaagaatttcctgaggcagatgatgatttaaaaagtaatctgaaggaaattatccttcaatgcctttcaacagattgaactactgtgtcttataggaagtaagtaatgcagtggtttggtgtttgactaaaatataagtgaaaactttcttttatatttatggcaacagaattttactttctaattagagatcacagaataagaaacatgtttaactcatattaaatctttatatattaaatctttataaatcaaccaaatagaaatgtctacaaggatggctggttctgggtagacttcaacattttcattcttagaagacttggatcctgagagaaaattgtaatcctatatcaatttgatgactaaagaagcacaggattaagattaaattagtaaaaaacccaggagactgattacaatcagacggaaggcatgcgatacctagtcttcctactcctttcccaaattcatctaatcggaacaaaagaaggagagaagagaattaaattatgaagagatgccaatacaattattttcatataaaataggtcaaaattatataagaataatgtgtaagattatacagctactaggaaatacagctgaattaaatgtaaacattttttcttaatcagctgtaaaacgacacaaaagcattgaaaagaatcacaagttcctttgtaaatctaggttccataaaaatgctatcctttgtgagtgaagaatggagaaaaaatccttactttacatactttaaaaaaattataaatgtgtacaaacaattctcatagtgtgatgacttaaaatttaaagttttgccacaatgaaaaccaacaagtgaatcactttttcaaaactttttctcaatcagaaaaaatgaggtacataaaagccaaaaagtcaaagacaaaaaacattatagggtctacattcttcttcatatatatttttttttataatttaagtcaagctaatgtacttatacaatttcatataaaaggaaaaataaaatgaatatccccaaatttgttctacaaattcaactacataaaatttgaggcatactctggtataacacatattaaagaaccaatacaatttaagagcataacctactttttaaaggttaattggatgaccgatttaaagactgtaccaaatgaacactggtctaattgcctattttgttgttattgctaaaaagaaatactaatgaagactgtaaccttgttttctatagcccccccaaattctaacaaaaccaaatggtatcagtagaacaatttatggatcaggcatggtggctcatgcttgtaatcccagtgctttaggaggccaggagttcaagaccagcctggtcaacatagtgagactcatctctacaaaaaattaaaaaaattaaaattaagccaggtgcagtgactcatgcctgtaatcctagcactttgggaggctgaggtgggcagatcacttgaggtcaggagtttgagaccaacatggcaaaactccatctccactaaaaatacaaaaactagctggatgtggtggcacgcacctgtagtcccagttactcgggaggctgagacagaagaatcacttgaacctgggaggtggaggttgcagtgagctgagattgtgccactgcactccagcctgggcaacaaagccagactccgtctcaaaaaaagaaaaaaaaattaaaattagccaggtgtagtggtgcatgcctacagtcttagctacttgggaggctgaagctggaggactgcttgagcctaggagttcaaggttataatgaactatgattatgccactgctctccagcctgtgtgacagagcaagaccctgtctctataaaaaatttttttaagtagaataatttatgggttacagagcattataataaatactatttcatttgatccttacaatatccagtgagggaggctaaaaccaaaaattaccttatccacattttacattgaagaaacaaagactcagagaaataaaatgaccagcccagttgacatcatgagtcttaaaattccaatcccaggggaattttcattacaccagactatgtaagtcatccaaatatggtaatatgtaaatgtacctttggcatgtcaaaaagcaatataaatatcatcataatgaaattttggtatgttaatattttctaagctccagcaaatgattcactaatttatataaaaaaaattaagtggttcctttcatttcacagagatatagcctaactaagatgggtacagtttgagttattttcagctattatcacaaagaaactgatgaggtaggttaaaatgtagtaaatttttctaatttgaagacattcttaggatttttataaatctgctctaagagcagcagaaaaagaaaggttgatttgaagattcatttactcagctggtccacaaagatctaacagcataagactaaaaggagtctaattactcacttctaagaatcactgttcatcttctaaaattaattaaaaggattggtacatgtctgtacatatatttctttaattataatagtgatatggactgttatctatgcaaaatatgtttcatttggtgtactttacatatttattacctgccacatattattctggtaaagcagagacttcatttcacataggttatagatctttcaaatttctttgatgtgagactcagtactagggtaaaagcaagttgtgtgacatgaattgttcatttaaatatttattgaaaaactgtgtatgaatccctgtgccagctgagttattaaccaattgttctttgaaacaaactgttttgagtttaatattatcttagatcttttgtctagttattgaataaaaaaagttgctgaaatcaaagtactttttgaaaaccttttgataatatattaacatgttagagagaactattattttctcagttgtcaactgaaaaaagaaaacactaaacattatcatatgccaatcaaagttaaacatatggtaggaaaactgtccagacttattcagattggtttaagctagttagacttaaaactgctgcccaaactgaatactgttgtttaaaaccatggattaatattacataaattttgtgggacaaaattaagatacttactgaaagtaactgaaaagtcaatatagtattcccatacatacccacaatttaatagagaaaatacaaatgattatctaaaaatctagaagcacaaagttaagattttcatagtgatgttcacttaactgtctatacttggcccacttgtaaaagaaaaccaattaacattttggcagttgataatataatgcagatggcaatggatgacaacatcttcgagcccaaactggtaccttctattttaacttatttttgtttgtgaatgtttgttttagttctctcatgctgtttgcaggagagattctcagacaaaagcttcatgaattattgataaataagttgttatatgtttggctttcagagaaaatgtttactaattgtcggttatgagggaattcagacctgcctgctttgagcattaactccagctccaaggagaaaggcaatgaacacagagaaaaatgaaaaacattttgggccaaatattcaaatatctctcatgaagaataagtcatattatcatacatgtactttgaaatatataacataatagacaaattattactatcagaaaactgactttgctgcctgatgagaatattctttttcaacacctaatttcttggcagtttgttttaaagggtaagaaagaaagtatacatgaattcaacacacgtcaaggaatgtactatagcagtcctcacacctcttaaatccacaataacctaatcccttatcattcataatgctttacagttttcaaagagctttcacataatttttttcacttgatcttaatctgacagctttgtgaggtaggtagagtacgtatttatcttctatcttcatttacaaacaagggaactgaggctcggagagttaaattgttaaaggtcataaactataatagcataaggcagagccaggcctcttcagagtctagaataattcttcaaagtatgattcttggattacctccgtaagaatcacctgcggtatttttataactacagattttaaagtcctatcactttggccttactgagtaagtctctctaggagtacagcccagaatttggcatcaggtgcagaacaactgaatattagataatgatataaaagcgaaagacagaatccatgtggatgttcatgtgatatatgatgccgacagatcatcaggggcaagttaaagtagtgagtttcaagccaggctgcagattagaatcacctggagcgctttttttttttttttttttttttaagaaagctaccaattcttatttgtatgagaggaaggtgttaggcatctgaagtaacccaagtgattcttatctgcagtcagggttgaggacccttgtttaaatatgctttttacataatacatcaagcatgttccagcatttttctttctcttctgattgatttcatgcctaataagttttacagtttatattgtaaattatttaaacattatcagataaacatttttacttgattttttaaagattaaatgatattcatactaagactaatcatgcttcatttagctacaacaattttcaaatactcaaatcaatcaccactttggactgaggttatatatatttcagttgtaaacaagaatgatccagaatctgaaaataagggtgtggggcaaaagctgtagcctactggctattgggcaaggcaagtgcagacaatcaactcactacaggagggcctggaagccaaggtctggtggctttggcaagatcacatctcactgtagaaaaatacaacaatgaatacagagaaaatgttttgccattttgtaattgtggttaccttataatgtatgatgtttatcttattacatgcctccacaaagcaaattttgaacattaagttctctatgaatcaatactattacatgggaaaagatggctacaaattaaaatttttccatcatgcatatggataagttataaaaacacagccagaaaaagtaatatttacaaaagttataaaaacagcacaattataggggaaacaatgcccatctctttattccactgctaatccaaaccctgaatatctctgcatgaagattatttcgatagaattttaagagaacctttcatagactaatcaaattcttctgttgcacttttattctattagctaaaatacccttgctgatttattaaattctcctacagtttaaaaacacagttcttttttcacttagtggaaataaaactacaaagtcctactgttcatctgagaagtaaaccttgcatagaaaatttctttaattctgaaattgttttattaactgagctaccagaatgttatctcacaactagtttatagtatatgaaagttcactacaaagcagtcaccacacatttaggatttttctaaatataaaatgagtgggtttataaaaatgcttaccagacaaataattatctcttcataacctagaaagacgaattatttttgtgatgatagaattcttagtgttttggatgccttgatgttccaagtttgatgcaatataaaaaagcaatcatttacctttccagtggacacaatctgtacttgactgaaagcatgttaactgtgagttacagctatcagtcatgcaaaaggcaaagaataaaatctgctttttaaacagcacaagatttccaccttagacaagacaaattaagcactggttccatcttcttcaataacccgattcatgctggtgccatgtgtgatatgagtcatgggattattactgagatctctgatgctgctatgtcgtgactgttcattgagccgatgagaactactatgcctggagtgatctgttagtcgtgacatgctgccatgaggtagtctctcctccattcctctgtaactgcagggcgtgtacctgccatcacgtgatctgtggaggctgccgtggtagctgctcactttgctgtggatgcttcctgctttgcttctttgatcatccaccatagccagctgagttgaagaagcatgggtggatgttccttgagtggaagttccccttgactttcttatgataggagtatttggatccctcaggagagactgagcaaaatcaggttcctggagtacctgtcggctctcattcactatctcttttttcctacgaccatgaaaaaaactggcccattcaaagcatgtctttttgcttccaacccaaaatacagagggaatgccaactatgagagccatcaggtatttcatcagaaagagaatcaagtctggacgactcatttgagtaacctgatatggacatggaatgtgatattctctgcagcgttcttgtatccacgttgtttcccagatgccccggtaagcttgctcataaaagtagcatccaattacaaccaagagtggtacgagataaagaatgctgaaaacaccgatccggatcataaacttcactaatttatcttggttctccttttctaatggaatctcaattcgaactctgtttagggatataatgccagctaagaggagagaaaccccaactaccacatacaggcagaggggagcaagaacaaaatatctcaatgcatcaacatcgtagaggccaacaaaacacacgccactaatattgtcaccttcaattttattcatcgctaaaaggatgatggttagagttccggggatgccccatgcactggcgtgaaacagcaatgctttcttctcaatagcttcactaccccactttggcacagctgctaaaaaccatgtgatggtaagaattacccaccatacactgccagccatagtaaaaaaatagagtatcataaaaagcatggtacaggctttattatgagatccttgtgtcactgtggaagccttatattgtgcagggatggatgcattgcaggctactcgatcttcaagcaaaaatccaatgaagaaaattaaggataccatcatgtagcagactgcataaaatataataggcctttcaggataacggaatcttgtgacatcaatcaaaaaagttaaaaaagtaaacaatgtggccgagaggcaaatgattgaaatcaatcctatgaaatagcgagcaaatgacagttcttctcttctgaagtacatatttggacaaggaggtgaacaatcacgcacatgcagaaaagaataacccagatcaggatcaatttttaactctcggggacaccaaaaaccatagtctctctgcactgccactggggctccttcagttggttctccagctaaattcagatccacaagtcgaggatatggctcatcacaatctgggaacctactgcattccatatcttcaggccaaggaacaccaaacatctccatgagcttcgaacactcactgtaagcccgctgacacagcctacgacagggaagtgtgacacgtccatattccatacaaataggagcgtagagtgcacaaagaaaaggccggaaatcccgagaacaatccagattcaccatagggtggaatggctccattgccaaagctgctgtctgttggtcataatgattcagaagattaggcatgaaggtagtattataaggcaaatcttggcacatcctcaaggtaataggttcacaagaaaacaaactgtgcccacctatatgccccatgaacacagtcaagggccaaagagagaagacaatccaagtcatagccatccttcctgggtctgaaggagattcagatgatcaggcctattcaatatgtattttagatatttatacacctgcaggtctcagctcgaaggtacttcttctgtatcttactgttaaattcttcaaacagttaaatactcttcgcaccgtcagaggtttgttagcttggtctcacaaaaggcgtttgtttttggtttcacaatatgggaaaatgacatcatcttgtctcttcttttcattttattacatggggcacatttggccaacatatcaagttgatcaaccacattcccaaaccacagattccatcttaggagaagagctatttcttccttcaactgaaatatctcagaccccggcgcctggctccaaggggtgggggggctgcaccgcctgccgcgggcggccgcgcgtccctcaggtacccggagcggccgaggaacgccggcgcgcgcctcccagcgacagcgagctttcgc

SEQ ID NO: 11352 - RNA, 10031 nt, Homo sapiens
  source 1..10031: mol_type = other RNA
ctgaatagctgggactacaggtgcccgccaccatgcccaactaatttttttgtttttagtagagacagggtctcaccatgttagccaggacggtcttgatctcctgacctcgtgatccgcccgcctcggcctcccaaagtgttgggattacaggcgtgagccactgcgcctggctaatttttgtatttttagtacagaaggggatttgccatgttcatcaggctggtctcgaactcctgacctcaggtgatctgcccaccttggcctcccaaagtgctgggattacaggcgtgagccactgcgtctggcctcaatctctacattatatcagatgacaattaaggaatttttccagaaacattttctgtatagccagaaaaaaattaaaaataacaagccacattgatctctaataatatttcaaatgaagacattcacttgcccatggcaatctggcaactatatttatgtaataaacctaagaatgcagtttaagaataattactgaacaaaaaattttcaatcaactcctctgaaatttcttttacattttataattattttaatattggtaaattgaattgcttttaaattagccatacgaaccattgctttgttcactaatttgatcttgaatacattttgtgtaaattttaggctaactagctatattcatatttaagagaacaaagaccacaaaacgttatgtcattcttttctatgtatcaatttaaggtgcttatattggtgcttaagaagactttcccatttaaaaaagccatgtccaatatttataactttctttcatttttattatctgtaatataattttccttctttaaaattacttaaaatcactaatggaaaaacagttgataaaatatctgaatcccatcaatttacatgtaaatgacgttaataatacaggttgatctagtaaaataatacaagttgatctagttcatgggatgaataagaagaataaaaatgagaccaaaataatgattataaaatggtcaaatgagaaccaaatgagagctgggcggaattttagacgctacctaaactaattctcttgttccctagagaatgagaaaaatggaggcaccacgagataaaatgccttatccaaagttacacagctaactgcaaaagagaggcaagagtagaagtcaagtttcctgactcaaaatcctattgtatttttaaaaataaaataatacagttttactaatcattaaaaaaatcctgccaatttagaaaatagatttttttgtttaattttagactccaggatagaaaatagaaattattaagctctaagttaaaaaaaaaaaccaataagcacaacacaaagaaatatctgcaatttagcatatacaaacaagctgacttatacaacaaaaaaccttaaagctacaataataataaagtaatccatcctactccaggaatatgataaaatatcaaccttaaaaaaactttaaaaactaactttactagttaatggtaattagcaaaataatgaaacagtgaatcttcaaaatctgaattatttcaaggtaaaaaacatttttaatctttatcgggaaaaactggtgacagtgaccaataaaatgagcataaagtataagcaacgctttcacaccaacaaaaaaattcaagaaagaatttcctgaggcagatgatgatttaaaaagtaatctgaaggaaattatccttcaatgcctttcaacagattgaactactgtgtcttataggaagtaagtaatgcagtggtttggtgtttgactaaaatataagtgaaaactttcttttatatttatggcaacagaattttactttctaattagagatcacagaataagaaacatgtttaactcatattaaatctttatatattaaatctttataaatcaaccaaatagaaatgtctacaaggatggctggttctgggtagacttcaacattttcattcttagaagacttggatcctgagagaaaattgtaatcctatatcaatttgatgactaaagaagcacaggattaagattaaattagtaaaaaacccaggagactgattacaatcagacggaaggcatgcgatacctagtcttcctactcctttcccaaattcatctaatcggaacaaaagaaggagagaagagaattaaattatgaagagatgccaatacaattattttcatataaaataggtcaaaattatataagaataatgtgtaagattatacagctactaggaaatacagctgaattaaatgtaaacattttttcttaatcagctgtaaaacgacacaaaagcattgaaaagaatcacaagttcctttgtaaatctaggttccataaaaatgctatcctttgtgagtgaagaatggagaaaaaatccttactttacatactttaaaaaaattataaatgtgtacaaacaattctcatagtgtgatgacttaaaatttaaagttttgccacaatgaaaaccaacaagtgaatcactttttcaaaactttttctcaatcagaaaaaatgaggtacataaaagccaaaaagtcaaagacaaaaaacattatagggtctacattcttcttcatatatatttttttttataatttaagtcaagctaatgtacttatacaatttcatataaaaggaaaaataaaatgaatatccccaaatttgttctacaaattcaactacataaaatttgaggcatactctggtataacacatattaaagaaccaatacaatttaagagcataacctactttttaaaggttaattggatgaccgatttaaagactgtaccaaatgaacactggtctaattgcctattttgttgttattgctaaaaagaaatactaatgaagactgtaaccttgttttctatagcccccccaaattctaacaaaaccaaatggtatcagtagaacaatttatggatcaggcatggtggctcatgcttgtaatcccagtgctttaggaggccaggagttcaagaccagcctggtcaacatagtgagactcatctctacaaaaaattaaaaaaattaaaattaagccaggtgcagtgactcatgcctgtaatcctagcactttgggaggctgaggtgggcagatcacttgaggtcaggagtttgagaccaacatggcaaaactccatctccactaaaaatacaaaaactagctggatgtggtggcacgcacctgtagtcccagttactcgggaggctgagacagaagaatcacttgaacctgggaggtggaggttgcagtgagctgagattgtgccactgcactccagcctgggcaacaaagccagactccgtctcaaaaaaagaaaaaaaaattaaaattagccaggtgtagtggtgcatgcctacagtcttagctacttgggaggctgaagctggaggactgcttgagcctaggagttcaaggttataatgaactatgattatgccactgctctccagcctgtgtgacagagcaagaccctgtctctataaaaaatttttttaagtagaataatttatgggttacagagcattataataaatactatttcatttgatccttacaatatccagtgagggaggctaaaaccaaaaattaccttatccacattttacattgaagaaacaaagactcagagaaataaaatgaccagcccagttgacatcatgagtcttaaaattccaatcccaggggaattttcattacaccagactatgtaagtcatccaaatatggtaatatgtaaatgtacctttggcatgtcaaaaagcaatataaatatcatcataatgaaattttggtatgttaatattttctaagctccagcaaatgattcactaatttatataaaaaaaattaagtggttcctttcatttcacagagatatagcctaactaagatgggtacagtttgagttattttcagctattatcacaaagaaactgatgaggtaggttaaaatgtagtaaatttttctaatttgaagacattcttaggatttttataaatctgctctaagagcagcagaaaaagaaaggttgatttgaagattcatttactcagctggtccacaaagatctaacagcataagactaaaaggagtctaattactcacttctaagaatcactgttcatcttctaaaattaattaaaaggattggtacatgtctgtacatatatttctttaattataatagtgatatggactgttatctatgcaaaatatgtttcatttggtgtactttacatatttattacctgccacatattattctggtaaagcagagacttcatttcacataggttatagatctttcaaatttctttgatgtgagactcagtactagggtaaaagcaagttgtgtgacatgaattgttcatttaaatatttattgaaaaactgtgtatgaatccctgtgccagctgagttattaaccaattgttctttgaaacaaactgttttgagtttaatattatcttagatcttttgtctagttattgaataaaaaaagttgctgaaatcaaagtactttttgaaaaccttttgataatatattaacatgttagagagaactattattttctcagttgtcaactgaaaaaagaaaacactaaacattatcatatgccaatcaaagttaaacatatggtaggaaaactgtccagacttattcagattggtttaagctagttagacttaaaactgctgcccaaactgaatactgttgtttaaaaccatggattaatattacataaattttgtgggacaaaattaagatacttactgaaagtaactgaaaagtcaatatagtattcccatacatacccacaatttaatagagaaaatacaaatgattatctaaaaatctagaagcacaaagttaagattttcatagtgatgttcacttaactgtctatacttggcccacttgtaaaagaaaaccaattaacattttggcagttgataatataatgcagatggcaatggatgacaacatcttcgagcccaaactggtaccttctattttaacttatttttgtttgtgaatgtttgttttagttctctcatgctgtttgcaggagagattctcagacaaaagcttcatgaattattgataaataagttgttatatgtttggctttcagagaaaatgtttactaattgtcggttatgagggaattcagacctgcctgctttgagcattaactccagctccaaggagaaaggcaatgaacacagagaaaaatgaaaaacattttgggccaaatattcaaatatctctcatgaagaataagtcatattatcatacatgtactttgaaatatataacataatagacaaattattactatcagaaaactgactttgctgcctgatgagaatattctttttcaacacctaatttcttggcagtttgttttaaagggtaagaaagaaagtatacatgaattcaacacacgtcaaggaatgtactatagcagtcctcacacctcttaaatccacaataacctaatcccttatcattcataatgctttacagttttcaaagagctttcacataatttttttcacttgatcttaatctgacagctttgtgaggtaggtagagtacgtatttatcttctatcttcatttacaaacaagggaactgaggctcggagagttaaattgttaaaggtcataaactataatagcataaggcagagccaggcctcttcagagtctagaataattcttcaaagtatgattcttggattacctccgtaagaatcacctgcggtatttttataactacagattttaaagtcctatcactttggccttactgagtaagtctctctaggagtacagcccagaatttggcatcaggtgcagaacaactgaatattagataatgatataaaagcgaaagacagaatccatgtggatgttcatgtgatatatgatgccgacagatcatcaggggcaagttaaagtagtgagtttcaagccaggctgcagattagaatcacctggagcgctttttttttttttttttttttttaagaaagctaccaattcttatttgtatgagaggaaggtgttaggcatctgaagtaacccaagtgattcttatctgcagtcagggttgaggacccttgtttaaatatgctttttacataatacatcaagcatgttccagcatttttctttctcttctgattgatttcatgcctaataagttttacagtttatattgtaaattatttaaacattatcagataaacatttttacttgattttttaaagattaaatgatattcatactaagactaatcatgcttcatttagctacaacaattttcaaatactcaaatcaatcaccactttggactgaggttatatatatttcagttgtaaacaagaatgatccagaatctgaaaataagggtgtggggcaaaagctgtagcctactggctattgggcaaggcaagtgcagacaatcaactcactacaggagggcctggaagccaaggtctggtggctttggcaagatcacatctcactgtagaaaaatacaacaatgaatacagagaaaatgttttgccattttgtaattgtggttaccttataatgtatgatgtttatcttattacatgcctccacaaagcaaattttgaacattaagttctctatgaatcaatactattacatgggaaaagatggctacaaattaaaatttttccatcatgcatatggataagttataaaaacacagccagaaaaagtaatatttacaaaagttataaaaacagcacaattataggggaaacaatgcccatctctttattccactgctaatccaaaccctgaatatctctgcatgaagattatttcgatagaattttaagagaacctttcatagactaatcaaattcttctgttgcacttttattctattagctaaaatacccttgctgatttattaaattctcctacagtttaaaaacacagttcttttttcacttagtggaaataaaactacaaagtcctactgttcatctgagaagtaaaccttgcatagaaaatttctttaattctgaaattgttttattaactgagctaccagaatgttatctcacaactagtttatagtatatgaaagttcactacaaagcagtcaccacacatttaggatttttctaaatataaaatgagtgggtttataaaaatgcttaccagacaaataattatctcttcataacctagaaagacgaattatttttgtgatgatagaattcttagtgttttggatgccttgatgttccaagtttgatgcaatataaaaaagcaatcatttacctttccagtggacacaatctgtacttgactgaaagcatgttaactgtgagttacagctatcagtcatgcaaaaggcaaagaataaaatctgctttttaaacagcacaagatttccaccttagacaagacaaattaagcactggttccatcttcttcaataacccgattcatgctggtgccatgtgtgatatgagtcatgggattattactgagatctctgatgctgctatgtcgtgactgttcattgagccgatgagaactactatgcctggagtgatctgttagtcgtgacatgctgccatgaggtagtctctcctccattcctctgtaactgcagggcgtgtacctgccatcacgtgatctgtggaggctgccgtggtagctgctcactttgctgtggatgcttcctgctttgcttctttgatcatccaccatagccagctgagttgaagaagcatgggtggatgttccttgagtggaagttccccttgactttcttatgataggagtatttggatccctcaggagagactgagcaaaatcaggttcctggagtacctgtcggctctcattcactatctcttttttcctacgaccatgaaaaaaactggcccattcaaagcatgtctttttgcttccaacccaaaatacagagggaatgccaactatgagagccatcaggtatttcatcagaaagagaatcaagtctggacgactcatttgagtaacctgatatggacatggaatgtgatattctctgcagcgttcttgtatccacgttgtttcccagatgccccggtaagcttgctcataaaagtagcatccaattacaaccaagagtggtacgagataaagaatgctgaaaacaccgatccggatcataaacttcactaatttatcttggttctccttttctaatggaatctcaattcgaactctgtttagggatataatgccagctaagaggagagaaaccccaactaccacatacaggcagaggggagcaagaacaaaatatctcaatgcatcaacatcgtagaggccaacaaaacacacgccactaatattgtcaccttcaattttattcatcgctaaaaggatgatggttagagttccggggatgccccatgcactggcgtgaaacagcaatgctttcttctcaatagcttcactaccccactttggcacagctgctaaaaaccatgtgatggtaagaattacccaccatacactgccagccatagtaaaaaaatagagtatcataaaaagcatggtacaggctttattatgagatccttgtgtcactgtggaagccttatattgtgcagggatggatgcattgcaggctactcgatcttcaagcaaaaatccaatgaagaaaattaaggataccatcatgtagcagactgcataaaatataataggcctttcaggataacggaatcttgtgacatcaatcaaaaaagttaaaaaagtaaacaatgtggccgagaggcaaatgattgaaatcaatcctatgaaatagcgagcaaatgacagttcttctcttctgaagtacatatttggacaaggaggtgaacaatcacgcacatgcagaaaagaataacccagatcaggatcaatttttaactctcggggacaccaaaaaccatagtctctctgcactgccactggggctccttcagttggttctccagctaaattcagatccacaagtcgaggatatggctcatcacaatctgggaacctactgcattccatatcttcaggccaaggaacaccaaacatctccatgagcttcgaacactcactgtaagcccgctgacacagcctacgacagggaagtgtgacacgtccatattccatacaaataggagcgtagagtgcacaaagaaaaggccggaaatcccgagaacaatccagattcaccatagggtggaatggctccattgccaaagctgctgtctgttggtcataatgattcagaagattaggcatgaaggtagtattataaggcaaatcttggcacatcctcaaggtaataggttcacaagaaaacaaactgtgcccacctatatgccccatgaacacagtcaagggccaaagagagaagacaatccaagtcatagccatccttcctgggtctgaaggagattcagatgatcaggcctattcaatatgtattttagatatttatacacctgcaggtctcagctcgaaggtacttcttctgtatcttactgttaaattcttcaaacagttaaatactcttcgcaccgtcagaggtttgttagcttggtctcacaaaaggcgtttgtttttggtttcacaatatgggaaaatgacatcatcttgtctcttcttttcattttattacatggggcacatttggccaacatatcaagttgatcaaccacattcccaaaccacagattccatcttaggagaagagctatttcttccttcaactgaaatatctcaggttacaagtgctccataagtcaggtcttgagaaatgctatcctcagaccccggcgcctggctccaaggggtgggggggctgcaccgcctgccgcgggcggccgcgcgtccctcaggtacccggagcggccgaggaacgccggcgcgcgcctcccagcgacagcgagctttcgc

SEQ ID NO: 11353 - RNA, 6503 nt, Homo sapiens
  source 1..6503: mol_type = other RNA
ctgaatagctgggactacaggtgcccgccaccatgcccggccaatttttgtatttttagtagagatggagtttcaccatactgtccaggctggtctcgaactcctgaccttgggatccgcctgccttggcctcccaaagtgctggtattacaggcatgagccaccacgcccggcctctcttttctattttattcatttattcactccatcactagagaacactggcttagagctgatgtgcctcagacacaggtgcactcatggagcacagaagcgagttggacaaagtccgggcctttgtagtgtgacgtggccattagggcccacagatccttccctgcagttgctgtctccctttcttcaggttccgaggaagccttccctggccgccttcataactctgacctcctccctccctccaacctaccagcatcaaatgcaccagctatgctcctcttttcccttgccgtctgttgccctgcactttgggaggctgaggcaggtggatcacccgaggtcgggagtttgagaccagcgtgaccaacatggagaaaacccatctctactaaaaatacaaaattagccgggcatggtggcatatgccaccactcttggagtgggcccaagaggaaaagatccctgcttatggccatgtcccagtgcctagaagagaggcggctcataggaagggttgaaaaaagtgtggaatgaatcaataaacagctcttgatttagtggcaggagaagtacaggcctcacctccaccgcgcaggcctcatctacgccatccagccctcacccacagtgtccagacctcacttctcccacccaggcctctacccagtcatctaggcattctccctgccgtctagcccaaaaccggaacagcacagccctcacctctgctgcccaggcctcatctacgccatccagccctcactcctgccgcccagccctcactcctgccgcccagccctcacctctgctgtccaggcatcacccttgctgtccagccgacacctacgatgcgcagtccatgtctccgctgcccaggcctcatctatgccacttagccctcacccatgccatctagccctcactcaagccacccagctctcacttcctccatccaggcatcattcctgccacccaggcctcatctacactgcctagccctcacctcccctgtccagcccgtcctcacctacactgcacagccctcacctctgccacccaggcctcatctatactgcccagccctcacctcccctgtccagccctcacctccccggtccagcccttgcctcccccgtccagccctcacctccatcatgcagccactgtctctgctgtccagtcctcacctatgccacattgtccgcatctacactgtacggccctcccctgtgccatccagctggcatcttctatgtaacacaacaagagctggaagagaagaggccctggtccctgggcgtggaggcgcagagccacccaggactgcaaaagaactcttaacggccaaccatggaactgggtgttgatatcccatggaacttgctaaactaggtgagcagaagagcactccaggccacccaaactgcgcggagaatccaggcacaaggaagtgctaagcagagccctcatgggctgtggggagtgggtggaggcactgccaacagggcaggagggattgagggaatgtccctgagccgccatactggggaggtgtgatctgggagcagagagccatggttggttacggagagtggcacaaacacggtgccagcgtccagcactgacagtcaggtggcgtggcagtcaatgcatggcccagatgggagactgaggcttgaactaagtcagtaatgagaaggataagctgaatataattcagaatactttcacaatttaggcaaaatttttttaaaaagtttccagttcactttgaggtttctacctggaataagcggatggtgatgtcattcaccgagatggaggcaaaagtttcggtggaaagataagatacctgggccaggcgcggtggctcacacctataatcctagcactctgggaggctgaggcaggcagatcacctgaggtcaggagttccagaccagcctggccaacacagtgaaaccccaactctactaaaaatacaaaaaatagccgggcatggtggcgtgcctagtcccagctactcgggaggctgaggcagaagaattgcttgaacccaggagacagaggttgcagtgagccgagatcgcaccactgcactccagcctgggcgacagagtgagactcagtctcaaaaaaaaaaaaaaagaaaagaaaagaaaagatatctagttctgaatatgatacaattgctactgttagttattcaagcgcataatgatctcccactactagcttggagagagggattgctttccaggtgacaaagcattgtcccctcccaggccaagagaaatgctcttgggtacagcaatagccctgctgagaaggggctggtctgaaggagtttcatgggaacctggttttcttgtctcgcttttacctatggtgtctttttccaccataagttccactcatccctgtggcctagtccacgggtcctcttttccatggtgccgcagagatgctccaggcagacgcctgctctggctgagacccgggccagctgcccctcctggctgctctccatcctgagatgcgcctgctcctttgtccccctgggagacacttgtacccccagctctgatcccagagcctggcctgctcctccttccacacatacgagcctgagaccccgctcacatgggaggcatttctcagtcacctccgcccagttacagcgagaaccgtgtggtcagagttgcatcttcctgagttgaatctggaaaatgcacgacctacttgtttaatgatgtaaaaacatgtgcttggatctgatctccatcactgaaccttaaacgcagagtcttccccttctgtctcctgcggctcataagtgccttatacttacatgatctgaggcaggttatcaaacgctcatgttctacctgctcctgagctctaggccaaaataggaatattaagagagccaagcatttgcttgtgctcatgttttgaaccatccagcccctcaccagtgccttcttccatttagctgacgtgacaatggcaggaaaccagcactccgcagcccatgcctcccaccaggatgctaccttgttggcgtccccatccgctctcaaatgctcacactcatataataaatacacgctacttaaaaaaaagaatggcttctttaaaaaccgcaaaggccagccgactgcagacagcctctgaagagctgctttccttgaccccccaaggctataaaataaatgcaatttgaataggaagtctgttcaaattcaccagctcctctgggaataatgaagataaaacccaagccttgatccctgtgttcgcaaaatgactcaaaaaaaaaaaaaaaaaaaaaaagaattgacatcatttaaaggactctgaggcttaagagtccaactctaaagtacacccactccctgaggacgcagagcaaatgcaggaaatcacgcccttccaggtgcaaaacaaatcagatcttgtccctctcacaggcatcaaaacacaaatcatcagttcccgacagaaacaaatcctgccctgccaagccaacagaaaaacactggagacagaaatgagctcagagaagggccgagggacaatgacaaggtggggaccctggacccttgggctccgctagccttccccacagcttgcagaagagggctcagctcctccattacagaagagacaaaatacagggactgcttccatcaaatcccccatcatctcactctgtctgtctgcagaagctgtcaggcctggctgggtgctgcctgtctcaggctcttactgcagagcttgtttccagagggccagaggccgtcctgtgtctcctttaatgcctgcgggggacgcagaggccactgagtctaggatcaggactgcgacacctactttctcaccgtcccatctgcctggtaaacctttgtctctctctgaacattctgcatttcagactgtcttgtagacaccatgaagtgaggttttggtttgagccaatttgaaaatctcttctttaaatgggcgagtaaagccgaatattcacaggcattgatacagctgttttttttttttttgtaaattatgctgacaatatggttattctaaggattaaatatttcacgtgttgaacacaatgcctggcacatagtaagttctattttaaatgtatattgaataaaacataaataggacgttaatgtgattaagacaaacagagaaaaggatttaaagagagaagaggccaggagacgcgggagaagacaatgctaacaggttgtcttaacaacacatggaaagctcctcactgcacagcccccagatgcctcactccacgagtgaaatccctgcacggcaggccgagagcgtgggtgcagcagtctgcctgacgtgagagccatgtcatcacatatctagaaggtaagggtacctccggttctggaacacacaatgtaggcacatttcgctgggggctccatgtacatttctaaatagataccagtgcagggacctggctaccctctgataagaaggaagtgaggcctgacagaaactgaccttccagtaacctggaagagactgctctgacggagacaggagatggctgctctgtgaatacacccaaatctcctagggcaggaggggcaaagtcaccgttctaggacacacctgtgaccacaccaggcctccaacaacggagcagctggctaaggaacgatgtcctggggctctggtcacatggaacagacccagtctgagctagagacaccccccaggcccaccaggcatcagcgtgggctcctgccatgcgtggagctcttcgtcttgacagggtccctgcgccaagaaggcaacaggctccgaggggaaaactcgagcaagagagtcccctgaatcggtgccatctgtctaaattccaagtatgcctgcctgatctaccagggcactgaagagtttaatagagaaaaaaaaaaacaatctgtgagctttatcccaagcacaaaacagccactcaggcgtgggagagctcctttctccccgtgtacgccacatgcactcactctacagggaccacaacatccaattcacaggcatggaggggaaacagcaaaataaacagacttcactttggagttgttttttagaaagctgcagtttgtgaatttctcttgctttttaaaacagaatatttccaaaacttgggcatcaatgcttggtctttttaggtgggggatagaagactgggccatcttcacagactctcagaccccggctctcggcggccccatttgccagccagacttcctgcttgggggacggctgctcccccggctcggtgcagttttgcagctgctggtcttgcttagtgaggcacagttctatctgaccaattgtctgtacttcctcatcctggcttggtggaaggcactggattttgggtatcactccatatactctggcaagggcatctttaaaatctgcaacttggtagtaattgatggatggttttatccccaattttagaagcacactgttgaggtccagctccctgtagagttccaggcttctgccaaagtacttcttctgggagttgagcgcatccacctgggcggcgcaggtcccatgcttttcccactcatgcttccagaagcggctgcgattgggaaacgagtgaattacgtcaggccagtatgccctcatttctggcaaaagatccttaatctcttctaaattgaagggccacgatctattacatccttcacttttatcgggccatagtccatgtattgtccagtaatccggagggtctctacagtcgttttgaattttctcgcatactgtctcaggccagtgctgaaccataattagttttttccactcatggttgtcacgcaggcgcttgtccgcaccgcccaggcaaagcaacgccaggcagaggcagcccagcagggccccgcgcagggctgcagggcgcatggtgccgacctgcggagagaacgctgccagctgccgctccggctcccacttcccacctgctgcccgaggaagacttccgggagaaacgctgtctccgagcccccgcgccgccgcgctccctccgctgcagcagcggccaccgggtgcgcccggagccctgggacggcctaaaccagtatctcgcgggccccgcgccgggctccgggaatggccgcagcagccctggcgacccgggcccctcggagctccccttcaggatcgtgcaccaagcgcgcacgtcccgggctctgcttcgcgacccacagcgaccccagctcctccacgctgcagccgccgtccgcccacgaccacggtcagtcgcgttgctc

SEQ ID NO: 11354 - RNA, 7222 nt, Homo sapiens
  source 1..7222: mol_type = other RNA
ctgaatagctgggactacaggtgcccgccaccatgcccggctaaatttttggatttttagtagaggcggggtgtcaccgtgttagccaggatagtctcgatctcctgacctcgtgatccacctgcctcagcctcccaaagtgctgggattacaggcgtgagccaccacgcccggcctttttttttttgagatggagtcttgctctgttgcccaggctggagtgcagtcatgtgatctccgctcactgcaagctctgccgcctgggttcgagcaattctcgtgcctcagcctcctgattagctgggattaaaggcatgtgccaatgtacctggctaattttttttgtatttttagtagagacggcgtttcaccatgttgaccaggcttgtctcaaactcctgacctcaggtgatacgcctcccttagccccccaagtgctgggattacaggtgtgagccaccgtgcccagcctcagcagcacatttctatttatagtttctaggtgatttattttctgcagactttcttgcatatggttaagcccaatcatttcatttaagttttataaacgtctgtattagaggatggcattttaaaattctttccccagaaccctggaatgtacctttctgggctatgcaagcctcatgcactgactacacagggccacatgggtaaatatatatgtattgatgtgtatttacatatcaaaaattaaatagactatatgcttaaattagaaacacaaagaacaaaggctaagttcactgctttactattcaataaaatagctttaaaaactgtgaaacagccaagtggccacattctaaacagcgacggagacctccaaaatattctgtccaccaaaaaaacacgaagtttctgaatatgtaaaaattagtagaaaatcaattaggtgacaaagtcattatagtagtggctttcaaaccctttataaaaaatagcagaatcattttaaatgtggaattattttatctactgagatctgaagcagcactcagtatacacaagtgtggctgcattgactgcagtgagaaggcaggcgcctccatggctcactgccccttggaggcgcactgcactaactcctgaagcaactccttgtcccccaacactgcatgggtcacagtccaaaaactgattccacatatgaatcataccaatttttatgtaacagagttcagacaaatatatcaatttgggtatgatacaaataagtttttcatagagttcttttagaaaagtgattttgagggaagaggacagcggagtagaagaaaaacaattttaagaacatacaattaattcaatttttcggcatggtatcccacctagcaaaagccctaggtgaatacatgaggttcagaccagaagctttcaaatttcagtatgcttaagaatcgcctgaggcgcttgttaataaaaacagagatttctatgttgcatctccagagacagggaatcattaagttaagggttgggctcaggaatccatactttcaacagcctgcccaggcattctgatgctgcagatagcctgcagcgcgtactctgaagaacaagagaaaggcttcaagggaaaaattgaaaaagacagggggacactgtttaaaagcaaaacccaaaccaccttttctgtcttgttgctgagaatgaattcagattgggataaacaaccttttctttctttttaaatatctagatattttaaatatatctacttatattccactgtcctcaactgggtagaaatattaaaaaaattatcaatataaaatgctggttcttgcttcaatattatcattttgaaggaaaaccacacaaaaccattacccattctaatgacttttttggccaaattatgtatttgggtccacattaatcattaaattagtataacctttaaagttttcaagttagtgcaaatttaaaattcaataaatatattaaatacaattttactttatattacaaatgtaaattatttttcttttgacatgctggtagtattcatttttacaacgcaaactgactttacaatttctgagtcacagtatattttataactctaagcaaatgtatttcacaaagcaaacactatatgtttttgacatactctaaaaaaataaaaataaataattttgattataaaatttgtataaacttagctacattaggggttcacagctaattgttgcagaaaacctaaaacacacctaaatcatgtaactttactagcagacaacttgtattttaaaacacaagtcagtttgatttctattaaacatgacgaaacactgaaaattatcatcatctgcctaagggatctttaagagctgccaggtattcagtatttaagccactacgtttataggaattaggaatgtattgggatagtaaaaagattagagaaatctggaaacagacatggagatatgatttacttcatgtatttcttcctgagaatgtagaagttatttttttaaatatcaagacaatttaaaatggaacaggaaaatcttatggcaattttttttggtaaagtgtagaatccctggtaatataaacaatcactaccctaatatgtaacttgcaaacatgaagtcttataaattgtacttaaacaaggcacatgcctatacacttatttgaaatgctgggtaaatgtgcccaaaaagtaagtgaattttgcaaaaacaagataatgatacattttatgagatggtattctgaaatagcttccctaaatgaagtctaaataagtgaataagccagcagaaaaacttcatgacagaccagtagtgatgcaaaaaccttactagattacaataaccaaaaaatcaacttatttagataaatgagggcattttacataagcctgttctaaatacagtgtaatattatggttggtattaaaattataatttttaattgtagttttcacaattaaaaagctgtattagttattgtgattattttcgttccaacatcctaaattgatttgcttctactacaattagcactacgaattatataacaggtaaactataacctacagcaaagtggatttaacagtgtatttataaaatgtgatgtctttaacaattttgatcatgaatgaaaggataaacttcataatactcagaacatgattggcccattaaaaaaaaaaaaaacaaaactctgccatcctcactgccatggttacttaccatgaaaggtatataaagaagctgaaaacagatctgctcacaaagtttctcaagactagaatttaagatcacctgaggagatctgcaagaggttaatttagcaaaatagagtatttcataaaatgtactgactactgtatacattactaagttgctctttgaaaacatggtctgggcctgaggtgaggcaaacttaggtttatggcaattcatggatgacagattcataatagaccctcaaagatagctaatggtattttgggggatacattctgatctttcagagattaatgtcatgaaagaccacaaagcctgggccatgtgtcagaaaaacaccaggctggatgccctctgggtcagccgacctgtgggtcacgacccttgggctggtcaacagcagcgaacaagcaccctctaatgggaaccatgaaactagcccttcagtaagtttgtggcaattgaggggcaaataaaacaatgaaacaaagctttcagttatccaaaagtagttccctagtgcttttcatgccctccttcatttttcaatacaatgaggaatatttgtgaagaataagaatatctagatttctgtcaggagaattaaattagaattttaattaatagactaaatttctatctgattgtgactagcagaatttatgtgatcaatttaacttattaaataaagctacagaacgtaaacactaaacacaggtaccataccacaaggtaaataataaataatttaaaaatatatctctctcattttaaaataaatatgatataaacattttagcaaagatttctgtccacttacctccctaaggggaaattctgttaaaagactactgtatttcaaaatactacaagaccaccaaatttttaaaacttatcagtcagccttgagctttttctaagcaattaatctcaccgttgtctcctttaagcacgttttttgaagtgttgacactgtcttttaataaaaagagcggctgataaacagttcagctcagaacctataacttacaatcccaagtgctctgaatcttatttcttaccaattcacttatctgtttctcttttggctacactggtgttataaaaaagatcctgaattgcagctcaaatggttacctacagaattaaacaacatttacgtgtctgaataagttcctaaaataaaaattgtaatacaaattttaagtatgatctttttttactattctccttttgggggttcctagaaatcaatacatacacttggtttgggttgtagaaaatcttaaggggcatgctgcaggaggatgctcacaattaaccatgctggtttgacagtaatcatttcctttcaaaaaagcaggttaatttgatctttccacccacaccttgttggagatataatgtgtccatccattgtgtgtccatcatatgcatggttcaaaaataagacatgagacagcacatacttcagagtgagtcccactctcaaaacagtcataacaaattttcactctcatgtaagtttttgtgactttttgtaagttaatactattcatttgaagtattttgctgaaaaaagaacaaacatttgtaaataactgaaggctggctggtttggggatgctatttacaaaaatgtatacccattatactactagtgaaattaagactgaatagctgatagagaatttctattaatacttttggatgaacatgtatctacttgcgtgaggattctatgcaaagttttcactccctcatccatctattcagtcgcctttatatcttcttgatccgaagtactagagatgtcatcatctgtttgttctccagagaaatataacatcattgcatgtgtcttgtgagttatggtgacagtgcagggcccttgggcccaaggctccccatccacctgcattggcatcatggagcacttcaaaatcagcctcactgtatgtgcctgtcctattcgaaaaggattagccagttttacttgaatctgagcacagtggaaagacccatatactccaacgacttccagcagaccatcgtcatgcctggctagagggtaagtctcgtcccccatcccttcccatagtctgcagccaccgccccagtatccgatgttcagaactataataccttccaagctgggcagtgctactcgctcaccatccagttctagctcaacttttttattcaaatctttacattcttgcactaaacaatctttggttccatagaataagtaaaccgccttattaagaattctgctagaaaacagagatggtgccttctcacgatgagcatgaaaattgagagccatgagagcatcaggtccaacagaaaaatagttgttcattgtgaattccttgggttttcttaagttgtagtatcctttatttgttacttgaactttccatcgatctagtttaattccatctgcttccattacatttcgcaaaacctgcgcaactggaatttctccagcataacctgtaccccaacccaatgtattggatagatcgttgcctgttcccagaggcaaaactgcaacttgtggaatgtacttttcttgtccccatgtaatcccagcactttgggaggccaaggtgggaggatcgcttgagcccaggagtttgacagcagcccaggcaacatggtgaaaccctgtctctacaaaaaatacaaaaattagccaggcatggtagcgcacacctatagtctcagcaactttgtaggctgaggtgggaggatggcttgaacctgagaaatggaggttgcagttagctgtgtctgcgccgctgcactccagcctgggtgacagtgcgagactgtatctcaagaaaaaacaacaacaacaacaaaacaacaacaaaacccatatatatatatatatgtatagtatatttatcttagaagtccttctgtagtagttcttaaagactaataccttaatcttcatgtcatcaactgcatccaggacccaccctacagtcccatcccctccacaaacaagtactcgagctgaataatatgggagaagagtacagagttgtagggctttgataggaggagttttagttacatcaaaaacctggactggattcaacaagatcctaaattctcccaacagtccttctcccatattagttccactacgagagttggccaggattattaatggggtccactgctttccaagcttagaggctagcacttcataatctgtttttttgtctttacgcatctgattaatggatgttaaataacttggtggaatgattaggtttttgaattctccaaaatcacatttttcattctttaaactatttttcatgcactcatcatgtactgttttctggcaccaaatgcacctgtaatcgcaaagcttgggttgacagccacactgctgcttgcaaaccatacagtaactgcacaggggcacgttgccccggatccagtggtggggcatggcgtccaggaccttggtgtcattcttgagcataatctccttgcactggaagcgcttgtcggccttcctgaggcagccctcgtccacgcggagcccgcagcagtcgcagaaggcgccctgcagaatgtgctgcgcgcacacgcagcagtaggtgggctggctgaacaggtccgtgtcgcgccacccgtgcttgctcttgcggaagatgtccctgcggtgcagctgccggcgcgaccgctggaggctacaccagaaggtgatgaacaccggcagcaggaccgagcacagcgtccacaagatcaggtgcccgtccgcaaacaggccctcggagggcgagcccggcgccggccgcctctccgcttccatcttctccaaggacgatacctcgcgcgggtggaggcgcggctccgggccagcaggccttggccgcctcgcgcaggaggagaacgacgctgggccgccagcagggatgaagccgggcgggggaaacgcttaaggctccagccgcacgcac

SEQ ID NO: 11355 - RNA, 6830 nt, Homo sapiens
  source 1..6830: mol_type = other RNA
ctgaatagctgggactacaggtgcccgccaccatgcccggctaaatttttggatttttagtagaggcggggtgtcaccgtgttagccaggatagtctcgatctcctgacctcgtgatccacctgcctcagcctcccaaagtgctgggattacaggcgtgagccaccacgcccggcctttttttttttgagatggagtcttgctctgttgcccaggctggagtgcagtcatgtgatctccgctcactgcaagctctgccgcctgggttcgagcaattctcgtgcctcagcctcctgattagctgggattaaaggcatgtgccaatgtacctggctaattttttttgtatttttagtagagacggcgtttcaccatgttgaccaggcttgtctcaaactcctgacctcaggtgatacgcctcccttagccccccaagtgctgggattacaggtgtgagccaccgtgcccagcctcagcagcacatttctatttatagtttctaggtgatttattttctgcagactttcttgcatatggttaagcccaatcatttcatttaagttttataaacgtctgtattagaggatggcattttaaaattctttccccagaaccctggaatgtacctttctgggctatgcaagcctcatgcactgactacacagggccacatgggtaaatatatatgtattgatgtgtatttacatatcaaaaattaaatagactatatgcttaaattagaaacacaaagaacaaaggctaagttcactgctttactattcaataaaatagctttaaaaactgtgaaacagccaagtggccacattctaaacagcgacggagacctccaaaatattctgtccaccaaaaaaacacgaagtttctgaatatgtaaaaattagtagaaaatcaattaggtgacaaagtcattatagtagtggctttcaaaccctttataaaaaatagcagaatcattttaaatgtggaattattttatctactgagatctgaagcagcactcagtatacacaagtgtggctgcattgactgcagtgagaaggcaggcgcctccatggctcactgccccttggaggcgcactgcactaactcctgaagcaactccttgtcccccaacactgcatgggtcacagtccaaaaactgattccacatatgaatcataccaatttttatgtaacagagttcagacaaatatatcaatttgggtatgatacaaataagtttttcatagagttcttttagaaaagtgattttgagggaagaggacagcggagtagaagaaaaacaattttaagaacatacaattaattcaatttttcggcatggtatcccacctagcaaaagccctaggtgaatacatgaggttcagaccagaagctttcaaatttcagtatgcttaagaatcgcctgaggcgcttgttaataaaaacagagatttctatgttgcatctccagagacagggaatcattaagttaagggttgggctcaggaatccatactttcaacagcctgcccaggcattctgatgctgcagatagcctgcagcgcgtactctgaagaacaagagaaaggcttcaagggaaaaattgaaaaagacagggggacactgtttaaaagcaaaacccaaaccaccttttctgtcttgttgctgagaatgaattcagattgggataaacaaccttttctttctttttaaatatctagatattttaaatatatctacttatattccactgtcctcaactgggtagaaatattaaaaaaattatcaatataaaatgctggttcttgcttcaatattatcattttgaaggaaaaccacacaaaaccattacccattctaatgacttttttggccaaattatgtatttgggtccacattaatcattaaattagtataacctttaaagttttcaagttagtgcaaatttaaaattcaataaatatattaaatacaattttactttatattacaaatgtaaattatttttcttttgacatgctggtagtattcatttttacaacgcaaactgactttacaatttctgagtcacagtatattttataactctaagcaaatgtatttcacaaagcaaacactatatgtttttgacatactctaaaaaaataaaaataaataattttgattataaaatttgtataaacttagctacattaggggttcacagctaattgttgcagaaaacctaaaacacacctaaatcatgtaactttactagcagacaacttgtattttaaaacacaagtcagtttgatttctattaaacatgacgaaacactgaaaattatcatcatctgcctaagggatctttaagagctgccaggtattcagtatttaagccactacgtttataggaattaggaatgtattgggatagtaaaaagattagagaaatctggaaacagacatggagatatgatttacttcatgtatttcttcctgagaatgtagaagttatttttttaaatatcaagacaatttaaaatggaacaggaaaatcttatggcaattttttttggtaaagtgtagaatccctggtaatataaacaatcactaccctaatatgtaacttgcaaacatgaagtcttataaattgtacttaaacaaggcacatgcctatacacttatttgaaatgctgggtaaatgtgcccaaaaagtaagtgaattttgcaaaaacaagataatgatacattttatgagatggtattctgaaatagcttccctaaatgaagtctaaataagtgaataagccagcagaaaaacttcatgacagaccagtagtgatgcaaaaaccttactagattacaataaccaaaaaatcaacttatttagataaatgagggcattttacataagcctgttctaaatacagtgtaatattatggttggtattaaaattataatttttaattgtagttttcacaattaaaaagctgtattagttattgtgattattttcgttccaacatcctaaattgatttgcttctactacaattagcactacgaattatataacaggtaaactataacctacagcaaagtggatttaacagtgtatttataaaatgtgatgtctttaacaattttgatcatgaatgaaaggataaacttcataatactcagaacatgattggcccattaaaaaaaaaaaaaacaaaactctgccatcctcactgccatggttacttaccatgaaaggtatataaagaagctgaaaacagatctgctcacaaagtttctcaagactagaatttaagatcacctgaggagatctgcaagaggttaatttagcaaaatagagtatttcataaaatgtactgactactgtatacattactaagttgctctttgaaaacatggtctgggcctgaggtgaggcaaacttaggtttatggcaattcatggatgacagattcataatagaccctcaaagatagctaatggtattttgggggatacattctgatctttcagagattaatgtcatgaaagaccacaaagcctgggccatgtgtcagaaaaacaccaggctggatgccctctgggtcagccgacctgtgggtcacgacccttgggctggtcaacagcagcgaacaagcaccctctaatgggaaccatgaaactagcccttcagtaagtttgtggcaattgaggggcaaataaaacaatgaaacaaagctttcagttatccaaaagtagttccctagtgcttttcatgccctccttcatttttcaatacaatgaggaatatttgtgaagaataagaatatctagatttctgtcaggagaattaaattagaattttaattaatagactaaatttctatctgattgtgactagcagaatttatgtgatcaatttaacttattaaataaagctacagaacgtaaacactaaacacaggtaccataccacaaggtaaataataaataatttaaaaatatatctctctcattttaaaataaatatgatataaacattttagcaaagatttctgtccacttacctccctaaggggaaattctgttaaaagactactgtatttcaaaatactacaagaccaccaaatttttaaaacttatcagtcagccttgagctttttctaagcaattaatctcaccgttgtctcctttaagcacgttttttgaagtgttgacactgtcttttaataaaaagagcggctgataaacagttcagctcagaacctataacttacaatcccaagtgctctgaatcttatttcttaccaattcacttatctgtttctcttttggctacactggtgttataaaaaagatcctgaattgcagctcaaatggttacctacagaattaaacaacatttacgtgtctgaataagttcctaaaataaaaattgtaatacaaattttaagtatgatctttttttactattctccttttgggggttcctagaaatcaatacatacacttggtttgggttgtagaaaatcttaaggggcatgctgcaggaggatgctcacaattaaccatgctggtttgacagtaatcatttcctttcaaaaaagcaggttaatttgatctttccacccacaccttgttggagatataatgtgtccatccattgtgtgtccatcatatgcatggttcaaaaataagacatgagacagcacatacttcagagtgagtcccactctcaaaacagtcataacaaattttcactctcatgtaagtttttgtgactttttgtaagttaatactattcatttgaagtattttgctgaaaaaagaacaaacatttgtaaataactgaaggctggctggtttggggatgctatttacaaaaatgtatacccattatactactagtgaaattaagactgaatagctgatagagaatttctattaatacttttggatgaacatgtatctacttgcgtgaggattctatgcaaagttttcactccctcatccatctattcagtcgcctttatatcttcttgatccgaagtactagagatgtcatcatctgtttgttctccagagaaatataacatcattgcatgtgtcttgtgagttatggtgacagtgcagggcccttgggcccaaggctccccatccacctgcattggcatcatggagcacttcaaaatcagcctcactgtatgtgcctgtcctattcgaaaaggattagccagttttacttgaatctgagcacagtggaaagacccatatactccaacgacttccagcagaccatcgtcatgcctggctagagggtaagtctcgtcccccatcccttcccatagtctgcagccaccgccccagtatccgatgttcagaactataataccttccaagctgggcagtgctactcgctcaccatccagttctagctcaacttttttattcaaatctttacattcttgcactaaacaatctttggttccatagaataagtaaaccgccttattaagaattctgctagaaaacagagatggtgccttctcacgatgagcatgaaaattgagagccatgagagcatcaggtccaacagaaaaatagttgttcattgtgaattccttgggttttcttaagttgtagtatcctttatttgttacttgaactttccatcgatctagtttaattccatctgcttccattacatttcgcaaaacctgcgcaactggaatttctccagcataacctgtaccccaacccaatgtattggatagatcgttgcctgttcccagaggcaaaactgcaacttgtggaatgtacttttcttgtcccttaatcttcatgtcatcaactgcatccaggacccaccctacagtcccatcccctccacaaacaagtactcgagctgaataatatgggagaagagtacagagttgtagggctttgataggaggagttttagttacatcaaaaacctggactggattcaacaagatcctaaattctcccaacagtccttctcccatattagttccactacgagagttggccaggattattaatggggtccactgctttccaagcttagaggctagcacttcataatctgtttttttgtctttacgcatctgattaatggatgttaaataacttggtggaatgattaggtttttgaattctccaaaatcacatttttcattctttaaactatttttcatgcactcatcatgtactgttttctggcaccaaatgcacctgtaatcgcaaagcttgggttgacagccacactgctgcttgcaaaccatacagtaactgcacaggggcacgttgccccggatccagtggtggggcatggcgtccaggaccttggtgtcattcttgagcataatctccttgcactggaagcgcttgtcggccttcctgaggcagccctcgtccacgcggagcccgcagcagtcgcagaaggcgccctgcagaatgtgctgcgcgcacacgcagcagtaggtgggctggctgaacaggtccgtgtcgcgccacccgtgcttgctcttgcggaagatgtccctgcggtgcagctgccggcgcgaccgctggaggctacaccagaaggtgatgaacaccggcagcaggaccgagcacagcgtccacaagatcaggtgcccgtccgcaaacaggccctcggagggcgagcccggcgccggccgcctctccgcttccatcttctccaaggacgatacctcgcgcgggtggaggcgcggctccgggccagcaggccttggccgcctcgcgcaggaggagaacgacgctgggccgccagcagggatgaagccgggcgggggaaacgctt

SEQ ID NO: 11356 - RNA, 6861 nt, Homo sapiens
  source 1..6861: mol_type = other RNA
ctgaatagctgggactacaggtgcccgccaccatgcccggctaaatttttggatttttagtagaggcggggtgtcaccgtgttagccaggatagtctcgatctcctgacctcgtgatccacctgcctcagcctcccaaagtgctgggattacaggcgtgagccaccacgcccggcctttttttttttgagatggagtcttgctctgttgcccaggctggagtgcagtcatgtgatctccgctcactgcaagctctgccgcctgggttcgagcaattctcgtgcctcagcctcctgattagctgggattaaaggcatgtgccaatgtacctggctaattttttttgtatttttagtagagacggcgtttcaccatgttgaccaggcttgtctcaaactcctgacctcaggtgatacgcctcccttagccccccaagtgctgggattacaggtgtgagccaccgtgcccagcctcagcagcacatttctatttatagtttctaggtgatttattttctgcagactttcttgcatatggttaagcccaatcatttcatttaagttttataaacgtctgtattagaggatggcattttaaaattctttccccagaaccctggaatgtacctttctgggctatgcaagcctcatgcactgactacacagggccacatgggtaaatatatatgtattgatgtgtatttacatatcaaaaattaaatagactatatgcttaaattagaaacacaaagaacaaaggctaagttcactgctttactattcaataaaatagctttaaaaactgtgaaacagccaagtggccacattctaaacagcgacggagacctccaaaatattctgtccaccaaaaaaacacgaagtttctgaatatgtaaaaattagtagaaaatcaattaggtgacaaagtcattatagtagtggctttcaaaccctttataaaaaatagcagaatcattttaaatgtggaattattttatctactgagatctgaagcagcactcagtatacacaagtgtggctgcattgactgcagtgagaaggcaggcgcctccatggctcactgccccttggaggcgcactgcactaactcctgaagcaactccttgtcccccaacactgcatgggtcacagtccaaaaactgattccacatatgaatcataccaatttttatgtaacagagttcagacaaatatatcaatttgggtatgatacaaataagtttttcatagagttcttttagaaaagtgattttgagggaagaggacagcggagtagaagaaaaacaattttaagaacatacaattaattcaatttttcggcatggtatcccacctagcaaaagccctaggtgaatacatgaggttcagaccagaagctttcaaatttcagtatgcttaagaatcgcctgaggcgcttgttaataaaaacagagatttctatgttgcatctccagagacagggaatcattaagttaagggttgggctcaggaatccatactttcaacagcctgcccaggcattctgatgctgcagatagcctgcagcgcgtactctgaagaacaagagaaaggcttcaagggaaaaattgaaaaagacagggggacactgtttaaaagcaaaacccaaaccaccttttctgtcttgttgctgagaatgaattcagattgggataaacaaccttttctttctttttaaatatctagatattttaaatatatctacttatattccactgtcctcaactgggtagaaatattaaaaaaattatcaatataaaatgctggttcttgcttcaatattatcattttgaaggaaaaccacacaaaaccattacccattctaatgacttttttggccaaattatgtatttgggtccacattaatcattaaattagtataacctttaaagttttcaagttagtgcaaatttaaaattcaataaatatattaaatacaattttactttatattacaaatgtaaattatttttcttttgacatgctggtagtattcatttttacaacgcaaactgactttacaatttctgagtcacagtatattttataactctaagcaaatgtatttcacaaagcaaacactatatgtttttgacatactctaaaaaaataaaaataaataattttgattataaaatttgtataaacttagctacattaggggttcacagctaattgttgcagaaaacctaaaacacacctaaatcatgtaactttactagcagacaacttgtattttaaaacacaagtcagtttgatttctattaaacatgacgaaacactgaaaattatcatcatctgcctaagggatctttaagagctgccaggtattcagtatttaagccactacgtttataggaattaggaatgtattgggatagtaaaaagattagagaaatctggaaacagacatggagatatgatttacttcatgtatttcttcctgagaatgtagaagttatttttttaaatatcaagacaatttaaaatggaacaggaaaatcttatggcaattttttttggtaaagtgtagaatccctggtaatataaacaatcactaccctaatatgtaacttgcaaacatgaagtcttataaattgtacttaaacaaggcacatgcctatacacttatttgaaatgctgggtaaatgtgcccaaaaagtaagtgaattttgcaaaaacaagataatgatacattttatgagatggtattctgaaatagcttccctaaatgaagtctaaataagtgaataagccagcagaaaaacttcatgacagaccagtagtgatgcaaaaaccttactagattacaataaccaaaaaatcaacttatttagataaatgagggcattttacataagcctgttctaaatacagtgtaatattatggttggtattaaaattataatttttaattgtagttttcacaattaaaaagctgtattagttattgtgattattttcgttccaacatcctaaattgatttgcttctactacaattagcactacgaattatataacaggtaaactataacctacagcaaagtggatttaacagtgtatttataaaatgtgatgtctttaacaattttgatcatgaatgaaaggataaacttcataatactcagaacatgattggcccattaaaaaaaaaaaaaacaaaactctgccatcctcactgccatggttacttaccatgaaaggtatataaagaagctgaaaacagatctgctcacaaagtttctcaagactagaatttaagatcacctgaggagatctgcaagaggttaatttagcaaaatagagtatttcataaaatgtactgactactgtatacattactaagttgctctttgaaaacatggtctgggcctgaggtgaggcaaacttaggtttatggcaattcatggatgacagattcataatagaccctcaaagatagctaatggtattttgggggatacattctgatctttcagagattaatgtcatgaaagaccacaaagcctgggccatgtgtcagaaaaacaccaggctggatgccctctgggtcagccgacctgtgggtcacgacccttgggctggtcaacagcagcgaacaagcaccctctaatgggaaccatgaaactagcccttcagtaagtttgtggcaattgaggggcaaataaaacaatgaaacaaagctttcagttatccaaaagtagttccctagtgcttttcatgccctccttcatttttcaatacaatgaggaatatttgtgaagaataagaatatctagatttctgtcaggagaattaaattagaattttaattaatagactaaatttctatctgattgtgactagcagaatttatgtgatcaatttaacttattaaataaagctacagaacgtaaacactaaacacaggtaccataccacaaggtaaataataaataatttaaaaatatatctctctcattttaaaataaatatgatataaacattttagcaaagatttctgtccacttacctccctaaggggaaattctgttaaaagactactgtatttcaaaatactacaagaccaccaaatttttaaaacttatcagtcagccttgagctttttctaagcaattaatctcaccgttgtctcctttaagcacgttttttgaagtgttgacactgtcttttaataaaaagagcggctgataaacagttcagctcagaacctataacttacaatcccaagtgctctgaatcttatttcttaccaattcacttatctgtttctcttttggctacactggtgttataaaaaagatcctgaattgcagctcaaatggttacctacagaattaaacaacatttacgtgtctgaataagttcctaaaataaaaattgtaatacaaattttaagtatgatctttttttactattctccttttgggggttcctagaaatcaatacatacacttggtttgggttgtagaaaatcttaaggggcatgctgcaggaggatgctcacaattaaccatgctggtttgacagtaatcatttcctttcaaaaaagcaggttaatttgatctttccacccacaccttgttggagatataatgtgtccatccattgtgtgtccatcatatgcatggttcaaaaataagacatgagacagcacatacttcagagtgagtcccactctcaaaacagtcataacaaattttcactctcatgtaagtttttgtgactttttgtaagttaatactattcatttgaagtattttgctgaaaaaagaacaaacatttgtaaataactgaaggctggctggtttggggatgctatttacaaaaatgtatacccattatactactagtgaaattaagactgaatagctgatagagaatttctattaatacttttggatgaacatgtatctacttgcgtgaggattctatgcaaagttttcactccctcatccatctattcagtcgcctttatatcttcttgatccgaagtactagagatgtcatcatctgtttgttctccagagaaatataacatcattgcatgtgtcttgtgagttatggtgacagtgcagggcccttgggcccaaggctccccatccacctgcattggcatcatggagcacttcaaaatcagcctcactgtatgtgcctgtcctattcgaaaaggattagccagttttacttgaatctgagcacagtggaaagacccatatactccaacgacttccagcagaccatcgtcatgcctggctagagggtaagtctcgtcccccatcccttcccatagtctgcagccaccgccccagtatccgatgttcagaactataataccttccaagctgggcagtgctactcgctcaccatccagttctagctcaacttttttattcaaatctttacattcttgcactaaacaatctttggttccatagaataagtaaaccgccttattaagaattctgctagaaaacagagatggtgccttctcacgatgagcatgaaaattgagagccatgagagcatcaggtccaacagaaaaatagttgttcattgtgaattccttgggttttcttaagttgtagtatcctttatttgttacttgaactttccatcgatctagtttaattccatctgcttccattacatttcgcaaaacctgcgcaactggaatttctccagcataacctgtaccccaacccaatgtattggatagatcgttgcctgttcccagaggcaaaactgcaacttgtggaatgtacttttcttgtcccttaatcttcatgtcatcaactgcatccaggacccaccctacagtcccatcccctccacaaacaagtactcgagctgaataatatgggagaagagtacagagttgtagggctttgataggaggagttttagttacatcaaaaacctggactggattcaacaagatcctaaattctcccaacagtccttctcccatattagttccactacgagagttggccaggattattaatggggtccactgctttccaagcttagaggctagcacttcataatctgtttttttgtctttacgcatctgattaatggatgttaaataacttggtggaatgattaggtttttgaattctccaaaatcacatttttcattctttaaactatttttcatgcactcatcatgtactgttttctggcaccaaatgcacctgtaatcgcaaagcttgggttgacagccacactgctgcttgcaaaccatacagtaactgcacaggggcacgttgccccggatccagtggtggggcatggcgtccaggaccttggtgtcattcttgagcataatctccttgcactggaagcgcttgtcggccttcctgaggcagccctcgtccacgcggagcccgcagcagtcgcagaaggcgccctgcagaatgtgctgcgcgcacacgcagcagtaggtgggctggctgaacaggtccgtgtcgcgccacccgtgcttgctcttgcggaagatgtccctgcggtgcagctgccggcgcgaccgctggaggctacaccagaaggtgatgaacaccggcagcaggaccgagcacagcgtccacaagatcaggtgcccgtccgcaaacaggccctcggagggcgagcccggcgccggccgcctctccgcttccatcttctccaaggacgataccttgccgccggtctgacccacggaagggcgcaacatacaggggcaagctgccctccaccgaaaggccgggcgttcaggccaggcaacgccggtcggcgcccgtaaccgtcggcccaggcctcgcactcccctccggggcgc

SEQ ID NO: 11357 - RNA, 7300 nt, Homo sapiens
  source 1..7300: mol_type = other RNA
ctgaatagctgggactacaggtgcccgccaccatgcccggctaaatttttggatttttagtagaggcggggtgtcaccgtgttagccaggatagtctcgatctcctgacctcgtgatccacctgcctcagcctcccaaagtgctgggattacaggcgtgagccaccacgcccggcctttttttttttgagatggagtcttgctctgttgcccaggctggagtgcagtcatgtgatctccgctcactgcaagctctgccgcctgggttcgagcaattctcgtgcctcagcctcctgattagctgggattaaaggcatgtgccaatgtacctggctaattttttttgtatttttagtagagacggcgtttcaccatgttgaccaggcttgtctcaaactcctgacctcaggtgatacgcctcccttagccccccaagtgctgggattacaggtgtgagccaccgtgcccagcctcagcagcacatttctatttatagtttctaggtgatttattttctgcagactttcttgcatatggttaagcccaatcatttcatttaagttttataaacgtctgtattagaggatggcattttaaaattctttccccagaaccctggaatgtacctttctgggctatgcaagcctcatgcactgactacacagggccacatgggtaaatatatatgtattgatgtgtatttacatatcaaaaattaaatagactatatgcttaaattagaaacacaaagaacaaaggctaagttcactgctttactattcaataaaatagctttaaaaactgtgaaacagccaagtggccacattctaaacagcgacggagacctccaaaatattctgtccaccaaaaaaacacgaagtttctgaatatgtaaaaattagtagaaaatcaattaggtgacaaagtcattatagtagtggctttcaaaccctttataaaaaatagcagaatcattttaaatgtggaattattttatctactgagatctgaagcagcactcagtatacacaagtgtggctgcattgactgcagtgagaaggcaggcgcctccatggctcactgccccttggaggcgcactgcactaactcctgaagcaactccttgtcccccaacactgcatgggtcacagtccaaaaactgattccacatatgaatcataccaatttttatgtaacagagttcagacaaatatatcaatttgggtatgatacaaataagtttttcatagagttcttttagaaaagtgattttgagggaagaggacagcggagtagaagaaaaacaattttaagaacatacaattaattcaatttttcggcatggtatcccacctagcaaaagccctaggtgaatacatgaggttcagaccagaagctttcaaatttcagtatgcttaagaatcgcctgaggcgcttgttaataaaaacagagatttctatgttgcatctccagagacagggaatcattaagttaagggttgggctcaggaatccatactttcaacagcctgcccaggcattctgatgctgcagatagcctgcagcgcgtactctgaagaacaagagaaaggcttcaagggaaaaattgaaaaagacagggggacactgtttaaaagcaaaacccaaaccaccttttctgtcttgttgctgagaatgaattcagattgggataaacaaccttttctttctttttaaatatctagatattttaaatatatctacttatattccactgtcctcaactgggtagaaatattaaaaaaattatcaatataaaatgctggttcttgcttcaatattatcattttgaaggaaaaccacacaaaaccattacccattctaatgacttttttggccaaattatgtatttgggtccacattaatcattaaattagtataacctttaaagttttcaagttagtgcaaatttaaaattcaataaatatattaaatacaattttactttatattacaaatgtaaattatttttcttttgacatgctggtagtattcatttttacaacgcaaactgactttacaatttctgagtcacagtatattttataactctaagcaaatgtatttcacaaagcaaacactatatgtttttgacatactctaaaaaaataaaaataaataattttgattataaaatttgtataaacttagctacattaggggttcacagctaattgttgcagaaaacctaaaacacacctaaatcatgtaactttactagcagacaacttgtattttaaaacacaagtcagtttgatttctattaaacatgacgaaacactgaaaattatcatcatctgcctaagggatctttaagagctgccaggtattcagtatttaagccactacgtttataggaattaggaatgtattgggatagtaaaaagattagagaaatctggaaacagacatggagatatgatttacttcatgtatttcttcctgagaatgtagaagttatttttttaaatatcaagacaatttaaaatggaacaggaaaatcttatggcaattttttttggtaaagtgtagaatccctggtaatataaacaatcactaccctaatatgtaacttgcaaacatgaagtcttataaattgtacttaaacaaggcacatgcctatacacttatttgaaatgctgggtaaatgtgcccaaaaagtaagtgaattttgcaaaaacaagataatgatacattttatgagatggtattctgaaatagcttccctaaatgaagtctaaataagtgaataagccagcagaaaaacttcatgacagaccagtagtgatgcaaaaaccttactagattacaataaccaaaaaatcaacttatttagataaatgagggcattttacataagcctgttctaaatacagtgtaatattatggttggtattaaaattataatttttaattgtagttttcacaattaaaaagctgtattagttattgtgattattttcgttccaacatcctaaattgatttgcttctactacaattagcactacgaattatataacaggtaaactataacctacagcaaagtggatttaacagtgtatttataaaatgtgatgtctttaacaattttgatcatgaatgaaaggataaacttcataatactcagaacatgattggcccattaaaaaaaaaaaaaacaaaactctgccatcctcactgccatggttacttaccatgaaaggtatataaagaagctgaaaacagatctgctcacaaagtttctcaagactagaatttaagatcacctgaggagatctgcaagaggttaatttagcaaaatagagtatttcataaaatgtactgactactgtatacattactaagttgctctttgaaaacatggtctgggcctgaggtgaggcaaacttaggtttatggcaattcatggatgacagattcataatagaccctcaaagatagctaatggtattttgggggatacattctgatctttcagagattaatgtcatgaaagaccacaaagcctgggccatgtgtcagaaaaacaccaggctggatgccctctgggtcagccgacctgtgggtcacgacccttgggctggtcaacagcagcgaacaagcaccctctaatgggaaccatgaaactagcccttcagtaagtttgtggcaattgaggggcaaataaaacaatgaaacaaagctttcagttatccaaaagtagttccctagtgcttttcatgccctccttcatttttcaatacaatgaggaatatttgtgaagaataagaatatctagatttctgtcaggagaattaaattagaattttaattaatagactaaatttctatctgattgtgactagcagaatttatgtgatcaatttaacttattaaataaagctacagaacgtaaacactaaacacaggtaccataccacaaggtaaataataaataatttaaaaatatatctctctcattttaaaataaatatgatataaacattttagcaaagatttctgtccacttacctccctaaggggaaattctgttaaaagactactgtatttcaaaatactacaagaccaccaaatttttaaaacttatcagtcagccttgagctttttctaagcaattaatctcaccgttgtctcctttaagcacgttttttgaagtgttgacactgtcttttaataaaaagagcggctgataaacagttcagctcagaacctataacttacaatcccaagtgctctgaatcttatttcttaccaattcacttatctgtttctcttttggctacactggtgttataaaaaagatcctgaattgcagctcaaatggttacctacagaattaaacaacatttacgtgtctgaataagttcctaaaataaaaattgtaatacaaattttaagtatgatctttttttactattctccttttgggggttcctagaaatcaatacatacacttggtttgggttgtagaaaatcttaaggggcatgctgcaggaggatgctcacaattaaccatgctggtttgacagtaatcatttcctttcaaaaaagcaggttaatttgatctttccacccacaccttgttggagatataatgtgtccatccattgtgtgtccatcatatgcatggttcaaaaataagacatgagacagcacatacttcagagtgagtcccactctcaaaacagtcataacaaattttcactctcatgtaagtttttgtgactttttgtaagttaatactattcatttgaagtattttgctgaaaaaagaacaaacatttgtaaataactgaaggctggctggtttggggatgctatttacaaaaatgtatacccattatactactagtgaaattaagactgaatagctgatagagaatttctattaatacttttggatgaacatgtatctacttgcgtgaggattctatgcaaagttttcactccctcatccatctattcagtcgcctttatatcttcttgatccgaagtactagagatgtcatcatctgtttgttctccagagaaatataacatcattgcatgtgtcttgtgagttatggtgacagtgcagggcccttgggcccaaggctccccatccacctgcattggcatcatggagcacttcaaaatcagcctcactgtatgtgcctgtcctattcgaaaaggattagccagttttacttgaatctgagcacagtggaaagacccatatactccaacgacttccagcagaccatcgtcatgcctggctagagggtaagtctcgtcccccatcccttcccatagtctgcagccaccgccccagtatccgatgttcagaactataataccttccaagctgggcagtgctactcgctcaccatccagttctagctcaacttttttattcaaatctttacattcttgcactaaacaatctttggttccatagaataagtaaaccgccttcggtgataagcaggaaatgttattttatccaacacaccttattaagaattctgctagaaaacagagatggtgccttctcacgatgagcatgaaaattgagagccatgagagcatcaggtccaacagaaaaatagttgttcattgtgaattccttgggttttcttaagttgtagtatcctttatttgttacttgaactttccatcgatctagtttaattccatctgcttccattacatttcgcaaaacctgcgcaactggaatttctccagcataacctgtaccccaacccaatgtattggatagatcgttgcctgttcccagaggcaaaactgcaacttgtggaatgtacttttcttgtccccatgtaatcccagcactttgggaggccaaggtgggaggatcgcttgagcccaggagtttgacagcagcccaggcaacatggtgaaaccctgtctctacaaaaaatacaaaaattagccaggcatggtagcgcacacctatagtctcagcaactttgtaggctgaggtgggaggatggcttgaacctgagaaatggaggttgcagttagctgtgtctgcgccgctgcactccagcctgggtgacagtgcgagactgtatctcaagaaaaaacaacaacaacaacaaaacaacaacaaaacccatatatatatatatatgtatagtatatttatcttagaagtccttctgtagtagttcttaaagactaataccttaatcttcatgtcatcaactgcatccaggacccaccctacagtcccatcccctccacaaacaagtactcgagctgaataatatgggagaagagtacagagttgtagggctttgataggaggagttttagttacatcaaaaacctggactggattcaacaagatcctaaattctcccaacagtccttctcccatattagttccactacgagagttggccaggattattaatggggtccactgctttccaagcttagaggctagcacttcataatctgtttttttgtctttacgcatctgattaatggatgttaaataacttggtggaatgattaggtttttgaattctccaaaatcacatttttcattctttaaactatttttcatgcactcatcatgtactgttttctggcaccaaatgcacctgtaatcgcaaagcttgggttgacagccacactgctgcttgcaaaccatacagtaactgcacaggggcacgttgccccggatccagtggtggggcatggcgtccaggaccttggtgtcattcttgagcataatctccttgcactggaagcgcttgtcggccttcctgaggcagccctcgtccacgcggagcccgcagcagtcgcagaaggcgccctgcagaatgtgctgcgcgcacacgcagcagtaggtgggctggctgaacaggtccgtgtcgcgccacccgtgcttgctcttgcggaagatgtccctgcggtgcagctgccggcgcgaccgctggaggctacaccagaaggtgatgaacaccggcagcaggaccgagcacagcgtccacaagatcaggtgcccgtccgcaaacaggccctcggagggcgagcccggcgccggccgcctctccgcttccatcttctccaaggacgataccttgccgccggtctgacccacggaagggcgcaacatacaggggcaagctgccctccaccgaaaggccgggcgttcaggccaggcaacgccggtcggcgcccgtaaccgtcggcccaggcctcgcactcccctccggggcgccgtctcctcccgggccccacccgctcc

SEQ ID NO: 11358 - RNA, 6792 nt, Homo sapiens
  source 1..6792: mol_type = other RNA
ctgaatagctgggactacaggtgcccgccaccatgcccggctaaatttttggatttttagtagaggcggggtgtcaccgtgttagccaggatagtctcgatctcctgacctcgtgatccacctgcctcagcctcccaaagtgctgggattacaggcgtgagccaccacgcccggcctttttttttttgagatggagtcttgctctgttgcccaggctggagtgcagtcatgtgatctccgctcactgcaagctctgccgcctgggttcgagcaattctcgtgcctcagcctcctgattagctgggattaaaggcatgtgccaatgtacctggctaattttttttgtatttttagtagagacggcgtttcaccatgttgaccaggcttgtctcaaactcctgacctcaggtgatacgcctcccttagccccccaagtgctgggattacaggtgtgagccaccgtgcccagcctcagcagcacatttctatttatagtttctaggtgatttattttctgcagactttcttgcatatggttaagcccaatcatttcatttaagttttataaacgtctgtattagaggatggcattttaaaattctttccccagaaccctggaatgtacctttctgggctatgcaagcctcatgcactgactacacagggccacatgggtaaatatatatgtattgatgtgtatttacatatcaaaaattaaatagactatatgcttaaattagaaacacaaagaacaaaggctaagttcactgctttactattcaataaaatagctttaaaaactgtgaaacagccaagtggccacattctaaacagcgacggagacctccaaaatattctgtccaccaaaaaaacacgaagtttctgaatatgtaaaaattagtagaaaatcaattaggtgacaaagtcattatagtagtggctttcaaaccctttataaaaaatagcagaatcattttaaatgtggaattattttatctactgagatctgaagcagcactcagtatacacaagtgtggctgcattgactgcagtgagaaggcaggcgcctccatggctcactgccccttggaggcgcactgcactaactcctgaagcaactccttgtcccccaacactgcatgggtcacagtccaaaaactgattccacatatgaatcataccaatttttatgtaacagagttcagacaaatatatcaatttgggtatgatacaaataagtttttcatagagttcttttagaaaagtgattttgagggaagaggacagcggagtagaagaaaaacaattttaagaacatacaattaattcaatttttcggcatggtatcccacctagcaaaagccctaggtgaatacatgaggttcagaccagaagctttcaaatttcagtatgcttaagaatcgcctgaggcgcttgttaataaaaacagagatttctatgttgcatctccagagacagggaatcattaagttaagggttgggctcaggaatccatactttcaacagcctgcccaggcattctgatgctgcagatagcctgcagcgcgtactctgaagaacaagagaaaggcttcaagggaaaaattgaaaaagacagggggacactgtttaaaagcaaaacccaaaccaccttttctgtcttgttgctgagaatgaattcagattgggataaacaaccttttctttctttttaaatatctagatattttaaatatatctacttatattccactgtcctcaactgggtagaaatattaaaaaaattatcaatataaaatgctggttcttgcttcaatattatcattttgaaggaaaaccacacaaaaccattacccattctaatgacttttttggccaaattatgtatttgggtccacattaatcattaaattagtataacctttaaagttttcaagttagtgcaaatttaaaattcaataaatatattaaatacaattttactttatattacaaatgtaaattatttttcttttgacatgctggtagtattcatttttacaacgcaaactgactttacaatttctgagtcacagtatattttataactctaagcaaatgtatttcacaaagcaaacactatatgtttttgacatactctaaaaaaataaaaataaataattttgattataaaatttgtataaacttagctacattaggggttcacagctaattgttgcagaaaacctaaaacacacctaaatcatgtaactttactagcagacaacttgtattttaaaacacaagtcagtttgatttctattaaacatgacgaaacactgaaaattatcatcatctgcctaagggatctttaagagctgccaggtattcagtatttaagccactacgtttataggaattaggaatgtattgggatagtaaaaagattagagaaatctggaaacagacatggagatatgatttacttcatgtatttcttcctgagaatgtagaagttatttttttaaatatcaagacaatttaaaatggaacaggaaaatcttatggcaattttttttggtaaagtgtagaatccctggtaatataaacaatcactaccctaatatgtaacttgcaaacatgaagtcttataaattgtacttaaacaaggcacatgcctatacacttatttgaaatgctgggtaaatgtgcccaaaaagtaagtgaattttgcaaaaacaagataatgatacattttatgagatggtattctgaaatagcttccctaaatgaagtctaaataagtgaataagccagcagaaaaacttcatgacagaccagtagtgatgcaaaaaccttactagattacaataaccaaaaaatcaacttatttagataaatgagggcattttacataagcctgttctaaatacagtgtaatattatggttggtattaaaattataatttttaattgtagttttcacaattaaaaagctgtattagttattgtgattattttcgttccaacatcctaaattgatttgcttctactacaattagcactacgaattatataacaggtaaactataacctacagcaaagtggatttaacagtgtatttataaaatgtgatgtctttaacaattttgatcatgaatgaaaggataaacttcataatactcagaacatgattggcccattaaaaaaaaaaaaaacaaaactctgccatcctcactgccatggttacttaccatgaaaggtatataaagaagctgaaaacagatctgctcacaaagtttctcaagactagaatttaagatcacctgaggagatctgcaagaggttaatttagcaaaatagagtatttcataaaatgtactgactactgtatacattactaagttgctctttgaaaacatggtctgggcctgaggtgaggcaaacttaggtttatggcaattcatggatgacagattcataatagaccctcaaagatagctaatggtattttgggggatacattctgatctttcagagattaatgtcatgaaagaccacaaagcctgggccatgtgtcagaaaaacaccaggctggatgccctctgggtcagccgacctgtgggtcacgacccttgggctggtcaacagcagcgaacaagcaccctctaatgggaaccatgaaactagcccttcagtaagtttgtggcaattgaggggcaaataaaacaatgaaacaaagctttcagttatccaaaagtagttccctagtgcttttcatgccctccttcatttttcaatacaatgaggaatatttgtgaagaataagaatatctagatttctgtcaggagaattaaattagaattttaattaatagactaaatttctatctgattgtgactagcagaatttatgtgatcaatttaacttattaaataaagctacagaacgtaaacactaaacacaggtaccataccacaaggtaaataataaataatttaaaaatatatctctctcattttaaaataaatatgatataaacattttagcaaagatttctgtccacttacctccctaaggggaaattctgttaaaagactactgtatttcaaaatactacaagaccaccaaatttttaaaacttatcagtcagccttgagctttttctaagcaattaatctcaccgttgtctcctttaagcacgttttttgaagtgttgacactgtcttttaataaaaagagcggctgataaacagttcagctcagaacctataacttacaatcccaagtgctctgaatcttatttcttaccaattcacttatctgtttctcttttggctacactggtgttataaaaaagatcctgaattgcagctcaaatggttacctacagaattaaacaacatttacgtgtctgaataagttcctaaaataaaaattgtaatacaaattttaagtatgatctttttttactattctccttttgggggttcctagaaatcaatacatacacttggtttgggttgtagaaaatcttaaggggcatgctgcaggaggatgctcacaattaaccatgctggtttgacagtaatcatttcctttcaaaaaagcaggttaatttgatctttccacccacaccttgttggagatataatgtgtccatccattgtgtgtccatcatatgcatggttcaaaaataagacatgagacagcacatacttcagagtgagtcccactctcaaaacagtcataacaaattttcactctcatgtaagtttttgtgactttttgtaagttaatactattcatttgaagtattttgctgaaaaaagaacaaacatttgtaaataactgaaggctggctggtttggggatgctatttacaaaaatgtatacccattatactactagtgaaattaagactgaatagctgatagagaatttctattaatacttttggatgaacatgtatctacttgcgtgaggattctatgcaaagttttcactccctcatccatctattcagtcgcctttatatcttcttgatccgaagtactagagatgtcatcatctgtttgttctccagagaaatataacatcattgcatgtgtcttgtgagttatggtgacagtgcagggcccttgggcccaaggctccccatccacctgcattggcatcatggagcacttcaaaatcagcctcactgtatgtgcctgtcctattcgaaaaggattagccagttttacttgaatctgagcacagtggaaagacccatatactccaacgacttccagcagaccatcgtcatgcctggctagagggtaagtctcgtcccccatcccttcccatagtctgcagccaccgccccagtatccgatgttcagaactataataccttccaagctgggcagtgctactcgctcaccatccagttctagcttattaagaattctgctagaaaacagagatggtgccttctcacgatgagcatgaaaattgagagccatgagagcatcaggtccaacagaaaaatagttgttcattgtgaattccttgggttttcttaagttgtagtatcctttatttgttacttgaactttccatcgatctagtttaattccatctgcttccattacatttcgcaaaacctgcgcaactggaatttctccagcataacctgtaccccaacccaatgtattggatagatcgttgcctgttcccagaggcaaaactgcaacttgtggaatgtacttttcttgtcccttaatcttcatgtcatcaactgcatccaggacccaccctacagtcccatcccctccacaaacaagtactcgagctgaataatatgggagaagagtacagagttgtagggctttgataggaggagttttagttacatcaaaaacctggactggattcaacaagatcctaaattctcccaacagtccttctcccatattagttccactacgagagttggccaggattattaatggggtccactgctttccaagcttagaggctagcacttcataatctgtttttttgtctttacgcatctgattaatggatgttaaataacttggtggaatgattaggtttttgaattctccaaaatcacatttttcattctttaaactatttttcatgcactcatcatgtactgttttctggcaccaaatgcacctgtaatcgcaaagcttgggttgacagccacactgctgcttgcaaaccatacagtaactgcacaggggcacgttgccccggatccagtggtggggcatggcgtccaggaccttggtgtcattcttgagcataatctccttgcactggaagcgcttgtcggccttcctgaggcagccctcgtccacgcggagcccgcagcagtcgcagaaggcgccctgcagaatgtgctgcgcgcacacgcagcagtaggtgggctggctgaacaggtccgtgtcgcgccacccgtgcttgctcttgcggaagatgtccctgcggtgcagctgccggcgcgaccgctggaggctacaccagaaggtgatgaacaccggcagcaggaccgagcacagcgtccacaagatcaggtgcccgtccgcaaacaggccctcggagggcgagcccggcgccggccgcctctccgcttccatcttctccaaggacgataccttgccgccggtctgacccacggaagggcgcaacatacaggggcaagctgccctccaccgaaaggccgggcgttcaggccaggcaacgccggtcggcgcccgtaaccgtcggcccaggcctcgcactcccctccggggcgccgt

SEQ ID NO: 11359 - RNA, 935 nt, Homo sapiens
  source 1..935: mol_type = other RNA
ctgaatagctgggactacaggtgcccgccaccatgcccggctaattttttgtattttagtagagacggggtttcaccatattggccaggctggtctcaaactccttacctggtgatccgtccgccttggcctcccaaagtgctgagattacaggcgtgagccaccgcgcccagccaactttcaattttattagctgagtttttagcacaacattattaacttttaaaaacaaacatgtttgttttgaaataggcaaaacaacaaaaatattttgttttggaaagtaaatttatatgatcctgtaaatgtgtatgatatttagtaaagaaaaataaagatgagttgccatcttggaagagcaggctcactgaacagcagtgcttgtttcctcctccttcagaagggtcacagttggtggctaggtaacccggagaagggttttcctggggtcatcataacttgttctcattcacatacctttatccgtattcttagctcattttgcttcaaagacttacttgcacaatactatggcatacaaggactctcccacatgaatcagccaggcaagccaatacccattgcacaggagggtgtgatggtggtccaccaagtactgagtgaaggggcccaggggcccaaggttctgataagggatactctgaggccagaagacaacccacgcgaagtagcccagccccaggactgtgaccagagagggcaagggtcttgctggacggaaataggcggtagccgcattgctggcctccgacttcaccatcctcttgaaaaacccagacacagagttggctgggagctccccagccgtccccgcccccatataagaaaagcctggctagccggtttctcagggccctgggcgcccgcccaagaccctggcggaccagtatgcttgctctcattgcggagtctgg

SEQ ID NO: 11360 - RNA, 1162 nt, Homo sapiens
  source 1..1162: mol_type = other RNA
ctgaatagctgggactacaggtgcccgccaccatgcccggctaattttttgtattttagtagagacggggtttcaccatattggccaggctggtctcaaactccttacctggtgatccgtccgccttggcctcccaaagtgctgagattacaggcgtgagccaccgcgcccagccaactttcaattttattagctgagtttttagcacaacattattaacttttaaaaacaaacatgtttgttttgaaataggcaaaacaacaaaaatattttgttttggaaagtaaatttatatgatcctgtaaatgtgtatgatatttagtaaagaaaaataaagatgagttgccatcttggaagagcaggctcactgaacagcagtgcttgtttcctcctccttcagaagggtcacagttggtggctaggtaacccggagaagggttttcctggggtcatcataacttgttctcattcacatacctttatccgtattcttagctcattttgcttgcacaatactatggcatacaaggactctcccacatgaatcagccaggcaagccaatacccattgcacaggagggtgtgatggtggtccaccaagtactgagtgaaggggcccaggggcccaaggttctgataagggatactctgaggccagaagacaacccacacagaccgaagaaactctgaacagtcatttgggtctccattcttggcttctattttctttctttcttttttttttgacagggtctcactccgctgctggggttttccacgcatctttctcgttatcctttaaacagattatttctcagccaaacaaacgtcgctctttttctaggtacagctttcttcttgcttccacacctatgtcagaacagttatagcctctttatcctcccttaccacttaaatcctacccatcctttagatttatccccgttttccaaacaattcctattggctcaaacattctgcttcggaagccctattctgacttggcaggcctatggcagtctgttaacttgactttccgcttcgtgagaggcttaggctcggataacccgttagtaaccatgcagaggtgaggacccaaagacaggaacactagaaagcagaaactatcctaagagcccaccgaatttccgcttacatgagt

SEQ ID NO: 11361 - RNA, 1143 nt, Homo sapiens
  source 1..1143: mol_type = other RNA
ctgaatagctgggactacaggtgcccgccaccatgcccggctaattttttgtattttagtagagacggggtttcaccatattggccaggctggtctcaaactccttacctggtgatccgtccgccttggcctcccaaagtgctgagattacaggcgtgagccaccgcgcccagccaactttcaattttattagctgagtttttagcacaacattattaacttttaaaaacaaacatgtttgttttgaaataggcaaaacaacaaaaatattttgttttggaaagtaaatttatatgatcctgtaaatgtgtatgatatttagtaaagaaaaataaagatgagttgccatcttggaagagcaggctcactgaacagcagtgcttgtttcctcctccttcagaagggtcacagttggtggctaggtaacccggagaagggttttcctggggtcatcataacttgttctcattcacatacctttatccgtattcttagctcattttgcttgcacaatactatggcatacaaggactctcccacatgaatcagccaggcaagccaatacccattgcacaggagggtgtgatggtggtccaccaagtactgagtgaaggggcccaggggcccaaggttctgataagggatactctgaggccagaagacaacccacgaagaaactctgaacagtcatttgggtctccattcttggcttctattttctttctttcttttttttttgacagggtctcactccgctgctggggttttccacgcatctttctcgttatcctttaaacagattatttctcagccaaacaaacgtcgctctttttctaggtacagctttcttcttgcttccacacctatgtcagaacagttatagcctctttatcctcccttaccacttaaatcctacccatcctttagatttatccccgttttccaaacaattcctattggctcaaacattctgcttcggaagccctattctgacttggcaggcctatggcagtctgttaacttgactttccgcttcgtgagaggcttaggctcggataacccgttagtaaccatgcagaggtgaggacccaaagacaggaacactagaaagcagaaactatcctaagagcccaccgaatttcc

SEQ ID NO: 11362 - RNA, 2180 nt, Homo sapiens
  source 1..2180: mol_type = other RNA
ctgaatagctgggactacaggtgcccgccaccatgcccggctctggtctagtttttttcttctttgaatcccgtagggcctcagtgctgtgcagcaagcacatagttaaaactgaagaaaaatttcttgaataaaagtagttaacgtttttattctttacttcaaggtatatctccatgaataacctaaatgatcccccaaattggaatatccggcctaattccagggcggatggtggtgatggaagcaggtggaattatgccctgttggttccaatgctgggattggctgcttttcgtaagtcatggttttcttaaaattagtgttttccaggctgagagtgtggagccccggtgagggaggcagcatggtgtgggagcctgaaggccgtgactttgggacctgccagggacagccgagttttatcccctgcagtgaaccgtgggcaaatcacttaagctctgagcctcagtcttcctgttcacaggagatggataatcatacttaacctcagcacactgcaaggattaagtcagccaaggcgtttagaagcattttgtgtggggtgggttttaataacttagttccctctgaaggctttgctgctctcaagtcggggaggaggttccttatttcaggtgccctcataaggactgctggggaacaaaacgggtgtaaaggaaaccagtgggctgggcgtggtggctcatacctgtaaccccagcactctgcgagacccaggtgggcagatcgagtgaccagcctgagcaacacagcaaaaccccgtctctacaaaaaatacaaaaattagcgagtcgtggcggtgcacacctgtagtcccagctactcaggaggctgaggtgggaagatcagtggagcctgggaggtcgaggctgcagtgagtggagatggcaccacttgccctccagcctgagaaacagggttaaaaaaaaaaaaagaaaaccagttttggaaaaccagtgatgtttaatgtttaggaaatcagtctttgggagacttcatccatgaaatctctgcttggcctggccagaaattctctctagtttagattgacttggcaccactttggggaactgtcagtcacatgcagacttacatccccaccacacaatcaattcactgatgcagaggagtgagttttgtgtttcttcacattccatggttctgggctggcacttaggaacatgagaaactgaataattgaatggaagaaaggcaagactgccctctagttgtagcgatacattttgtgtagcggctttttatctgcttcgatgtctcaggtcagaagttttgctgtagaggaagaggaggctggtaagagcaggtggtttttatgattcagtgatctgcgcagtgcttgcttcttggtgaaagacagggcaggtccacatccaatcctaaggggctgccatgtaaaaagctcatccgcctgcaggcttgggaaaaaaacccttaacacttggagaggctactgttgcctgtggctagggtgagtggattggaaggcttaaaattactctgactaatgtaataattaattggctttgaggctgggagaggccctgaagtgactcattttccatttgtttttcagactcatctcaagcttttatagcctttcatgataactttcacttctgaaattcttaccttcccttcttggacttttgaaatgatgctttctgtccctgaaaagggttgaagaatattttttcttcctggttttttgctgaggtagtgtggtcagagataactgttaacttggtgttcttgtaaggattctccaaaggtgtgttacgatgtgtttgaggttctattgcacataagagcgtaaccagccttcagtgtagtatatgatcgacctgacagtcactggattaaagggagtccacgtgccgttggagagagcttgctgaagctcggtgtctgatatcactccactcctgtctttatcgaccctctggaagacgttccacaggaagctctggtcgggcagcgccgcgcccgcagcaggcccagggccgcccggggctggggcggtaggagtaggcagccaagggccaaggcccgccgctgggctgaagcgcctgcggcgactggcgacccctcagagcgacaccgcttccgcctctgctgggggcagggccgggcgttac

SEQ ID NO: 11363 - RNA, 1845 nt, Homo sapiens
  source 1..1845: mol_type = other RNA
ctgaatagctgggactacaggtgcccgccaccatgcctggctaatgttttgtatttttagtacagacggggtttcaccatgttggccaggctggtctcaaactcctgacctcaagtgatccacctgccttggcttcccaaagtgcaaggattacaggcgtgagtcactgcgcctggccatatggagcactttctatgtgccatgcactaagtctcaagtataaggcaggaaaaaaaaaaaaacaaaaaaaaaaagggacagaaatcctgcctttgcagagttttcattctggtgattatttctaccacgtattactggtatggtaaaagtgatcagcaactaacaaaactagcagggttaaaatgactagaatgtgtaatgagctaaaattgacagggaaaaaaaacaggtatcactaataacaaaatttaaatctacaaaatttgatccagacgattttcacttaatagaaagaatggccacaaaagaatcaaacacacaaacaagaaaacctctccaaatagcagaagtcagaatcagcaaaaagatggtatataaaaagagactgatgagtcaaatgcctgttgtaaatttaaacagaaaataattgatcccatgaaaataatgttactacaaatagacattctaatggaaaaaaaatggaaatgattgagtcgagctgtataaaaaattaaactctggattaaaatggcttaatgaaatttgctctgcaaaacaggttgttccaaaaaattaatgtcacaagaattctcgcatggatgtttgcattaaagatgtacaaaaggctgaaacaatggggtaaaaattgaggaaggtacacaatagtcttcatctgtgtcatataatgcattgatagacacagccctaggctagtcagtgaggatatgagagctttttggagcactagcagcatcagattggagtgtgatgagaagctgctgacttagcctctctgccccatcctttttaagtgttactgtgtatctaagttacaatcttgttaaaatgcagattttgatgcagcaggtctggttctctcagaagattctgcatttctaacaagctcccaggtgatgcagatgctgcctcgtctgcagaccacactttgaggtctcttctgacactttgtgctgggatgacagctgctcaggggctggagcagtcctcaccactcccagcccttggatcacctgccttctttgcatggtctctccctggaaaggtggctggcgtggtcttgcatacttccaaaatctgcaatgcaactcgatcgccaggtcccgagcccttaatgagccagcccttgatgtgagtgtcaatcctgccatttgccttggtttgaccctcactccccaatcagggaatgttcagggatttactaatataatcctcttcatgattgcacgggaagagagcaaggcttaatctaagggaaggaatcactaggagtagaagcagtctggtgaggtaaaacaagtctagactccgaaagctgcgagttctccattcaaatgctgactcttccacttacaggtcttaggaaagccaggtgtccctttgggccttagttttctcatcttagtgtctggaggatcgtcatgggcatcctacaagacagcctcatagaagccagttctgcatggcttgggagtcctcaggaaagttacaatcatggtggaaggcacctcttcacagggcggcaggaagggtaagtgctgagccaagggggaggaaccccttataaaaccatcagatcttgtgagactcactcactttcgagagaagagcatgggggaaactgcccccatgattcaattacctcca

SEQ ID NO: 11364 - RNA, 3373 nt, Homo sapiens
  source 1..3373: mol_type = other RNA
ctgaatagctgggactacaggtgcccgccaccatgcctggctaattttttgtatttttagtagagatggggtctcaccatgttcgccaggatggtctcgatctcctgacctcgtgatccacccgcctcggcctcccaaagtgctgggattacaggcgtgagccaccgtgcccggccggtgacttctctttaaggatgaggcttatttcgcagaagagggcaagttccccacaaagggagctcttatgggaaagctaagggtataaagtctaaactaaacatatctttgataagtgttgtgcatcttagaaaagagaggttctggaatggtgactacatacacgcttctttgtgtttggggagagagtcacagaacagaccaaagggaaggctaagtggtctcttatcctggggatctggacggcgtgctgaagcctgaatttacactgatgtgttttagacagggaaacttaggagacatcgtaggcctgatactttgttatgattgatgcccttctgtttctctcctgggacaggtagtagatgcggttggcctctgggtaggtgactttgctgagcgggagcttgtagatggcggggttattggtcgtcaggagcaggaaggtgagagctgagagacagaagggccaagtgcagggcggcaatccaaacacagataacatgttagccagggcagcacccaggtaggcagcaaacagtgcgcaggcgatggcgaggaggtgcgtctgccaggtgatgacgtagaacatgcctcctatcgctatgcatgcgagggtgctgttgaagccacacaggccgaagtagatggagtcaaagggcgtcgcaatagtgagtgctgctagcatccccatggtggatccaattgctgcatgcaagcaaatgagaggtgaggatatgaacagagctatgaggaagatgcctccagtccaggggttatcacagccgtacacttggccaattccaacggggatggctctcaaaagcaagggcacttggacctctgaccaggtgatgttgggcatggcggatgcaggctgcagcagcgttgtggggaagaaaaggttgtagtggcccgtggctgccaggtacaaagtcacagtgatattgaagggcagtgtgaagactgggaggtcccacttgctgaagatggtacccagggcactggagaggatggggcaagacatggacatgatgatgacgggtagcaacagccaccagtagtagtcacctttgtctgagaacacggccatcagcagccccaccagcaccccattgtagccgtgaaatcctgcagcgatggccgacttgtcctgactcaggatgagggctgtcaaggtggacatgatggtacccaggcagcctgagatcgcccaccaggggttctggatgaagaggccgaggatgatgaggatgccgctgagggggttgttcacaaacatcacttgagatgtgcctcggaggacccagtcaaagaactggaacactggggacttgtctttaagtccctctccacactccttcatctctcctgtgatgtagctgagggctttgctgacccttttcccactggcagccatggaactccgaatccaggatgtcttggaaatgtttgtttccacttttatctcagagctctcctccatggtgtccagatcaagcagctcgactgtgggcttccggtatcgatagggaaatgggtctttgttttgtctttcctggtgttcgccttttccaaacactttgctcctcctccgaatggatgaccactcgatgtgaaatacactcctgtgcttggagagcacagcctccgagccctcctccacctttgggcctgctgtgggtggatgctccccaccgcctccgctgggggccttctcttcttcaccgcttttcactgtcaggtagtagatgcggttggcctcggggtaggtgactttgctgagtgggagtctgaagatggctgggttgtttgtcgtcaggagcaggaagatgatggtggcaaggcagaaggcccaggtgcctggtggcacgcccaccactgacatgatgttggagatggctgcttccatgtatgcacagaacagggcacagatgagggccagcaggtgagtctgccaggtgagggcatagaacatgcctccgatggcgatgcaggagaggacgcagttgtagctccagaggcctgtgtagatggtctcgaagggtgtggccactgacagggctgctagcagccccacgattgagccaatggctgcatgcaagcagatgagtggcgaggagatgaacagagccaccaggaacacgccgcctgtccagggattgtcacagccatacacctggccgaccccaacagggatggcttgtaacagcaggggcatttccatctctgtccaggtgatattgggcactgaagacacaggctctaccagtgttgtggggaagaagaggttgtagtggcctgtggctgcaaggtacaaggtgactgcaatgttgaagggcagagtgaagaccgggaggtcccacttgctgaagatggaattcaaggcactagaaagaactgggcaggacatggctgtgaaggtcacaggaaacagaagccaccagtagtagtctaacttctccgagaacacggccatcagcagtcccaccagcatcccgttgtacccatggagtcctgaggcaatggcagacctgtcttggcccaaggcgagagctgttaaggtcgagaccactgtccccaggcccccagtgattgtccaccagggattctggatcagcagccctatgaagatgatgaggccgctgagaggattgttgatgaacatcacctgagcggtccctctcaggacccagtctatgaactggagggcaaggtgcttgtctttcagccagatcctgtactccttcatgtcgcccgtgaggtagcccactgctttggagaggcagatgcacctttggcctgctgagtcccgatgggccaccccgtcgtctttccttttactcctttcattgagcttttcgatcttcacaatgtgactgtcttcattggaagaccggagatccttttcttcaggcatttccaggaggggcagagctgggtgagtatccggggatgtcgagggccagctcgggctggtaaactctgcctcgtagagtttgtatctgctggaaagtggctctggcaggagaggactgctgtgggggtcagacattccttcgggtcacagccactcttctatcgatggaacttccacattgctggggaggcctcaggaaacttacagtcatggtggaaggcgaaggggaagcaaacttggaccttctcaaatggcggcagaagagagagatggtgt

SEQ ID NO: 11365 - RNA, 3617 nt, Homo sapiens
  source 1..3617: mol_type = other RNA
ctgaatagctgggactacaggtgcccgccaccatgcctggctaattttttgtatttttagtagagatggggtctcaccatgttcgccaggatggtctcgatctcctgacctcgtgatccacccgcctcggcctcccaaagtgctgggattacaggcgtgagccaccgtgcccggccggtgacttctctttaaggatgaggcttatttcgcagaagagggcaagttccccacaaagggagctcttatgggaaagctaagggtataaagtctaaactaaacatatctttgataagtgttgtgcatcttagaaaagagaggttctggaatggtgactacatacacgcttctttgtgtttggggagagagtcacagaacagaccaaagggaaggctaagtggtctcttatcctggggatctggacggcgtgctgaagcctgaatttacactgatgtgttttagacagggaaacttaggagacatcgtaggcctgatactttgttatgattgatgcccttctgtttctctcctgggacaggtagtagatgcggttggcctctgggtaggtgactttgctgagcgggagcttgtagatggcggggttattggtcgtcaggagcaggaaggtgagagctgagagacagaagggccaagtgcagggcggcaatccaaacacagataacatgttagccagggcagcacccaggtaggcagcaaacagtgcgcaggcgatggcgaggaggtgcgtctgccaggtgatgacgtagaacatgcctcctatcgctatgcatgcgagggtgctgttgaagccacacaggccgaagtagatggagtcaaagggcgtcgcaatagtgagtgctgctagcatccccatggtggatccaattgctgcatgcaagcaaatgagaggtgaggatatgaacagagctatgaggaagatgcctccagtccaggggttatcacagccgtacacttggccaattccaacggggatggctctcaaaagcaagggcacttggacctctgaccaggtgatgttgggcatggcggatgcaggctgcagcagcgttgtggggaagaaaaggttgtagtggcccgtggctgccaggtacaaagtcacagtgatattgaagggcagtgtgaagactgggaggtcccacttgctgaagatggtacccagggcactggagaggatggggcaagacatggacatgatgatgacgggtagcaacagccaccagtagtagtcacctttgtctgagaacacggccatcagcagccccaccagcaccccattgtagccgtgaaatcctgcagcgatggccgacttgtcctgactcaggatgagggctgtcaaggtggacatgatggtacccaggcagcctgagatcgcccaccaggggttctggatgaagaggccgaggatgatgaggatgccgctgagggggttgttcacaaacatcacttgagatgtgcctcggaggacccagtcaaagaactggaacactggggacttgtctttaagtccctctccacactccttcatctctcctgtgatgtagctgagggctttgctgacccttttcccactggcagccatggaactccgaatccaggatgtcttggaaatgtttgtttccacttttatctcagagctctcctccatggtgtccagatcaagcagctcgactgtgggcttccggtatcgatagggaaatgggtctttgttttgtctttcctggtgttcgccttttccaaacactttgctcctcctccgaatggatgaccactcgatgtgaaatacactcctgtgcttggagagcacagcctccgagccctcctccacctttgggcctgctgtgggtggatgctccccaccgcctccgctgggggccttctcttcttcaccgcttttcactgtcaggtagtagatgcggttggcctcggggtaggtgactttgctgagtgggagtctgaagatggctgggttgtttgtcgtcaggagcaggaagatgatggtggcaaggcagaaggcccaggtgcctggtggcacgcccaccactgacatgatgttggagatggctgcttccatgtatgcacagaacagggcacagatgagggccagcaggtgagtctgccaggtgagggcatagaacatgcctccgatggcgatgcaggagaggacgcagttgtagctccagaggcctgtgtagatggtctcgaagggtgtggccactgacagggctgctagcagccccacgattgagccaatggctgcatgcaagcagatgagtggcgaggagatgaacagagccaccaggaacacgccgcctgtccagggattgtcacagccatacacctggccgaccccaacagggatggcttgtaacagcaggggcatttccatctctgtccaggtgatattgggcactgaagacacaggctctaccagtgttgtggggaagaagaggttgtagtggcctgtggctgcaaggtacaaggtgactgcaatgttgaagggcagagtgaagaccgggaggtcccacttgctgaagatggaattcaaggcactagaaagaactgggcaggacatggctgtgaaggtcacaggaaacagaagccaccagtagtagtctaacttctccgagaacacggccatcagcagtcccaccagcatcccgttgtacccatggagtcctgaggcaatggcagacctgtcttggcccaaggcgagagctgttaaggtcgagaccactgtccccaggcccccagtgattgtccaccagggattctggatcagcagccctatgaagatgatgaggccgctgagaggattgttgatgaacatcacctgagcggtccctctcaggacccagtctatgaactggagggcaaggtgcttgtctttcagccagatcctgtactccttcatgtcgcccgtgaggtagcccactgctttggagaggcagatgcacctttggcctgctgagtcccgatgggccaccccgtcgtctttccttttactcctttcattgagcttttcgatcttcacaatgtgactgtcttcattggaagaccggagatccttttcttcaggcatttccaggaggggcagagctgggtgagtatccggggatgtcgagggccagctcgggctggtaaactctgcctcgtagagtttgtatctgctggaaagtggctctggcaggagaggactgctgtgggggtcagacattccttcgggtcacagccactcttctatcgatggaagtttccttggtcacagtgttgtcagtggttctataaaggtcttatgaatctctacttagttgaccacaagtagtaagcaagaaacaatcggtcattcaggtcctgttggcacaatgaatggaggtgctccaagccttttccttgtctgtaggtagaggtgcaaatacttcaatgagatatgttcctgttcagaaacacccaggatgaaaactggaaagggtatttcctatggaggtgttctgagcaaagctgagggagctgatacccaaggcaggtatttcctcactcagccaactctcctcctccctctttcttcatacaaacttctctcttcatgcaacattagcata

SEQ ID NO: 11366 - RNA, 3920 nt, Homo sapiens
  source 1..3920: mol_type = other RNA
ctgaatagctgggactacaggtgcccgccaccatgcctggctaattttttgtatttttagtagagatggggtctcaccatgttcgccaggatggtctcgatctcctgacctcgtgatccacccgcctcggcctcccaaagtgctgggattacaggcgtgagccaccgtgcccggccggtgacttctctttaaggatgaggcttatttcgcagaagagggcaagttccccacaaagggagctcttatgggaaagctaagggtataaagtctaaactaaacatatctttgataagtgttgtgcatcttagaaaagagaggttctggaatggtgactacatacacgcttctttgtgtttggggagagagtcacagaacagaccaaagggaaggctaagtggtctcttatcctggggatctggacggcgtgctgaagcctgaatttacactgatgtgttttagacagggaaacttaggagacatcgtaggcctgatactttgttatgattgatgcccttctgtttctctcctgggacaggtagtagatgcggttggcctctgggtaggtgactttgctgagcgggagcttgtagatggcggggttattggtcgtcaggagcaggaaggtgagagctgagagacagaagggccaagtgcagggcggcaatccaaacacagataacatgttagccagggcagcacccaggtaggcagcaaacagtgcgcaggcgatggcgaggaggtgcgtctgccaggtgatgacgtagaacatgcctcctatcgctatgcatgcgagggtgctgttgaagccacacaggccgaagtagatggagtcaaagggcgtcgcaatagtgagtgctgctagcatccccatggtggatccaattgctgcatgcaagcaaatgagaggtgaggatatgaacagagctatgaggaagatgcctccagtccaggggttatcacagccgtacacttggccaattccaacggggatggctctcaaaagcaagggcacttggacctctgaccaggtgatgttgggcatggcggatgcaggctgcagcagcgttgtggggaagaaaaggttgtagtggcccgtggctgccaggtacaaagtcacagtgatattgaagggcagtgtgaagactgggaggtcccacttgctgaagatggtacccagggcactggagaggatggggcaagacatggacatgatgatgacgggtagcaacagccaccagtagtagtcacctttgtctgagaacacggccatcagcagccccaccagcaccccattgtagccgtgaaatcctgcagcgatggccgacttgtcctgactcaggatgagggctgtcaaggtggacatgatggtacccaggcagcctgagatcgcccaccaggggttctggatgaagaggccgaggatgatgaggatgccgctgagggggttgttcacaaacatcacttgagatgtgcctcggaggacccagtcaaagaactggaacactggggacttgtctttaagtccctctccacactccttcatctctcctgtgatgtagctgagggctttgctgacccttttcccactggcagccatggaactccgaatccaggatgtcttggaaatgtttgtttccacttttatctcagagctctcctccatggtgtccagatcaagcagctcgactgtgggcttccggtatcgatagggaaatgggtctttgttttgtctttcctggtgttcgccttttccaaacactttgctcctcctccgaatggatgaccactcgatgtgaaatacactcctgtgcttggagagcacagcctccgagccctcctccacctttgggcctgctgtgggtggatgctccccaccgcctccgctgggggccttctcttcttcaccgcttttcactgtcaggtagtagatgcggttggcctcggggtaggtgactttgctgagtgggagtctgaagatggctgggttgtttgtcgtcaggagcaggaagatgatggtggcaaggcagaaggcccaggtgcctggtggcacgcccaccactgacatgatgttggagatggctgcttccatgtatgcacagaacagggcacagatgagggccagcaggtgagtctgccaggtgagggcatagaacatgcctccgatggcgatgcaggagaggacgcagttgtagctccagaggcctgtgtagatggtctcgaagggtgtggccactgacagggctgctagcagccccacgattgagccaatggctgcatgcaagcagatgagtggcgaggagatgaacagagccaccaggaacacgccgcctgtccagggattgtcacagccatacacctggccgaccccaacagggatggcttgtaacagcaggggcatttccatctctgtccaggtgatattgggcactgaagacacaggctctaccagtgttgtggggaagaagaggttgtagtggcctgtggctgcaaggtacaaggtgactgcaatgttgaagggcagagtgaagaccgggaggtcccacttgctgaagatggaattcaaggcactagaaagaactgggcaggacatggctgtgaaggtcacaggaaacagaagccaccagtagtagtctaacttctccgagaacacggccatcagcagtcccaccagcatcccgttgtacccatggagtcctgaggcaatggcagacctgtcttggcccaaggcgagagctgttaaggtcgagaccactgtccccaggcccccagtgattgtccaccagggattctggatcagcagccctatgaagatgatgaggccgctgagaggattgttgatgaacatcacctgagcggtccctctcaggacccagtctatgaactggagggcaaggtgcttgtctttcagccagatcctgtactccttcatgtcgcccgtgaggtagcccactgctttggagaggcagatgcacctttggcctgctgagtcccgatgggccaccccgtcgtctttccttttactcctttcattgagcttttcgatcttcacaatgtgactgtcttcattggaagaccggagatccttttcttcaggcatttccaggaggggcagagctgggtgagtatccggggatgtcgagggccagctcgggctggtaaactctgcctcgtagagtttgtatctgctggaaagtggctctggcaggagaggactgctgtgggggtcagacattccttcgggtcacagccactcttctatcgatggaagtttccttggtcacagtgttgtcagtggttctataaaggtcttatgaatctctacttagttgaccacaagtagtaagcaagaaacaatcggtcattcaggtcctgttggcacaatgaatggaggtgctccaagccttttccttgtctgtaggtagaggtgcaaatacttcaatgagatatgttcctgttcagaaacacccaggatgaaaactggaaagggtcccacagttccgcctgaaccttgaagtgatggttttgagaagagtagtcaatatcacctaggagatcacactgggtaagaatgtggagtccttctcaggtgatcaaggcaaagaagacagccgactttgaaggcacataggtgtccaggggcttgttttcctggctcactctcctggctcactcagtccttccccactccttagtccctcagcactaacgtgggtctgtcatttcaggagatttgcttttgaagtgcctctcctcggactactctcattagcatcccgttctctttcaatggccaagtgatatgtgaggacctgattattttgccattggagaatttgcttcttaagtagccagacaacccaactcagcggccccagccagaaccactggaacggtgattcttcctgtgaccactctggttc

SEQ ID NO: 11367 - RNA, 3553 nt, Homo sapiens
  source 1..3553: mol_type = other RNA
ctgaatagctgggactacaggtgcccgccaccatgcctggctaattttttgtatttttagtagagatggggtctcaccatgttcgccaggatggtctcgatctcctgacctcgtgatccacccgcctcggcctcccaaagtgctgggattacaggcgtgagccaccgtgcccggccggtgacttctctttaaggatgaggcttatttcgcagaagagggcaagttccccacaaagggagctcttatgggaaagctaagggtataaagtctaaactaaacatatctttgataagtgttgtgcatcttagaaaagagaggttctggaatggtgactacatacacgcttctttgtgtttggggagagagtcacagaacagaccaaagggaaggctaagtggtctcttatcctggggatctggacggcgtgctgaagcctgaatttacactgatgtgttttagacagggaaacttaggagacatcgtaggcctgatactttgttatgattgatgcccttctgtttctctcctgggacaggtagtagatgcggttggcctctgggtaggtgactttgctgagcgggagcttgtagatggcggggttattggtcgtcaggagcaggaaggtgagagctgagagacagaagggccaagtgcagggcggcaatccaaacacagataacatgttagccagggcagcacccaggtaggcagcaaacagtgcgcaggcgatggcgaggaggtgcgtctgccaggtgatgacgtagaacatgcctcctatcgctatgcatgcgagggtgctgttgaagccacacaggccgaagtagatggagtcaaagggcgtcgcaatagtgagtgctgctagcatccccatggtggatccaattgctgcatgcaagcaaatgagaggtgaggatatgaacagagctatgaggaagatgcctccagtccaggggttatcacagccgtacacttggccaattccaacggggatggctctcaaaagcaagggcacttggacctctgaccaggtgatgttgggcatggcggatgcaggctgcagcagcgttgtggggaagaaaaggttgtagtggcccgtggctgccaggtacaaagtcacagtgatattgaagggcagtgtgaagactgggaggtcccacttgctgaagatggtacccagggcactggagaggatggggcaagacatggacatgatgatgacgggtagcaacagccaccagtagtagtcacctttgtctgagaacacggccatcagcagccccaccagcaccccattgtagccgtgaaatcctgcagcgatggccgacttgtcctgactcaggatgagggctgtcaaggtggacatgatggtacccaggcagcctgagatcgcccaccaggggttctggatgaagaggccgaggatgatgaggatgccgctgagggggttgttcacaaacatcacttgagatgtgcctcggaggacccagtcaaagaactggaacactggggacttgtctttaagtccctctccacactccttcatctctcctgtgatgtagctgagggctttgctgacccttttcccactggcagccatggaactccgaatccaggatgtcttggaaatgtttgtttccacttttatctcagagctctcctccatggtgtccagatcaagcagctcgactgtgggcttccggtatcgatagggaaatgggtctttgttttgtctttcctggtgttcgccttttccaaacactttgctcctcctccgaatggatgaccactcgatgtgaaatacactcctgtgcttggagagcacagcctccgagccctcctccacctttgggcctgctgtgggtggatgctccccaccgcctccgctgggggccttctcttcttcaccgcttttcactgtcaggtagtagatgcggttggcctcggggtaggtgactttgctgagtgggagtctgaagatggctgggttgtttgtcgtcaggagcaggaagatgatggtggcaaggcagaaggcccaggtgcctggtggcacgcccaccactgacatgatgttggagatggctgcttccatgtatgcacagaacagggcacagatgagggccagcaggtgagtctgccaggtgagggcatagaacatgcctccgatggcgatgcaggagaggacgcagttgtagctccagaggcctgtgtagatggtctcgaagggtgtggccactgacagggctgctagcagccccacgattgagccaatggctgcatgcaagcagatgagtggcgaggagatgaacagagccaccaggaacacgccgcctgtccagggattgtcacagccatacacctggccgaccccaacagggatggcttgtaacagcaggggcatttccatctctgtccaggtgatattgggcactgaagacacaggctctaccagtgttgtggggaagaagaggttgtagtggcctgtggctgcaaggtacaaggtgactgcaatgttgaagggcagagtgaagaccgggaggtcccacttgctgaagatggaattcaaggcactagaaagaactgggcaggacatggctgtgaaggtcacaggaaacagaagccaccagtagtagtctaacttctccgagaacacggccatcagcagtcccaccagcatcccgttgtacccatggagtcctgaggcaatggcagacctgtcttggcccaaggcgagagctgttaaggtcgagaccactgtccccaggcccccagtgattgtccaccagggattctggatcagcagccctatgaagatgatgaggccgctgagaggattgttgatgaacatcacctgagcggtccctctcaggacccagtctatgaactggagggcaaggtgcttgtctttcagccagatcctgtactccttcatgtcgcccgtgaggtagcccactgctttggagaggcagatgcacctttggcctgctgagtcccgatgggccaccccgtcgtctttccttttactcctttcattgagcttttcgatcttcacaatgtgactgtcttcattggaagaccggagatccttttcttcaggcatttccaggaggggcagagctgggtgagtatccggggatgtcgagggccagctcgggctggtaaactctgcctcgtagagtttgtatctgctggaaagtggctctggcaggagaggactgctgtgggggtcagacattccttcgggtcacagccactcttctatcgatggaagtttccttggtcacagtgttgtcagtggttctataaaggtcttatgaatctctacttagttgaccacaagtagtaagcaagaaacaatcggtcattcaggtcctgttggcacaatgaatggaggtgctccaagccttttccttgtctgtaggtagaggtgcaaatacttcaatgagatatgttcctgttcagaaacacccaggatgaaaactggaaagggtctgccaagaaatacagaggagctctttcagcatggtcgttttttaggatgatggaggcagcttac

SEQ ID NO: 11368 - RNA, 3949 nt, Homo sapiens
  source 1..3949: mol_type = other RNA
ctgaatagctgggactacaggtgcccgccaccatgcctggctaattttttgtatttttagtagagatggggtctcaccatgttcgccaggatggtctcgatctcctgacctcgtgatccacccgcctcggcctcccaaagtgctgggattacaggcgtgagccaccgtgcccggccggtgacttctctttaaggatgaggcttatttcgcagaagagggcaagttccccacaaagggagctcttatgggaaagctaagggtataaagtctaaactaaacatatctttgataagtgttgtgcatcttagaaaagagaggttctggaatggtgactacatacacgcttctttgtgtttggggagagagtcacagaacagaccaaagggaaggctaagtggtctcttatcctggggatctggacggcgtgctgaagcctgaatttacactgatgtgttttagacagggaaacttaggagacatcgtaggcctgatactttgttatgattgatgcccttctgtttctctcctgggacaggtagtagatgcggttggcctctgggtaggtgactttgctgagcgggagcttgtagatggcggggttattggtcgtcaggagcaggaaggtgagagctgagagacagaagggccaagtgcagggcggcaatccaaacacagataacatgttagccagggcagcacccaggtaggcagcaaacagtgcgcaggcgatggcgaggaggtgcgtctgccaggtgatgacgtagaacatgcctcctatcgctatgcatgcgagggtgctgttgaagccacacaggccgaagtagatggagtcaaagggcgtcgcaatagtgagtgctgctagcatccccatggtggatccaattgctgcatgcaagcaaatgagaggtgaggatatgaacagagctatgaggaagatgcctccagtccaggggttatcacagccgtacacttggccaattccaacggggatggctctcaaaagcaagggcacttggacctctgaccaggtgatgttgggcatggcggatgcaggctgcagcagcgttgtggggaagaaaaggttgtagtggcccgtggctgccaggtacaaagtcacagtgatattgaagggcagtgtgaagactgggaggtcccacttgctgaagatggtacccagggcactggagaggatggggcaagacatggacatgatgatgacgggtagcaacagccaccagtagtagtcacctttgtctgagaacacggccatcagcagccccaccagcaccccattgtagccgtgaaatcctgcagcgatggccgacttgtcctgactcaggatgagggctgtcaaggtggacatgatggtacccaggcagcctgagatcgcccaccaggggttctggatgaagaggccgaggatgatgaggatgccgctgagggggttgttcacaaacatcacttgagatgtgcctcggaggacccagtcaaagaactggaacactggggacttgtctttaagtccctctccacactccttcatctctcctgtgatgtagctgagggctttgctgacccttttcccactggcagccatggaactccgaatccaggatgtcttggaaatgtttgtttccacttttatctcagagctctcctccatggtgtccagatcaagcagctcgactgtgggcttccggtatcgatagggaaatgggtctttgttttgtctttcctggtgttcgccttttccaaacactttgctcctcctccgaatggatgaccactcgatgtgaaatacactcctgtgcttggagagcacagcctccgagccctcctccacctttgggcctgctgtgggtggatgctccccaccgcctccgctgggggccttctcttcttcaccgcttttcactgtcaggtagtagatgcggttggcctcggggtaggtgactttgctgagtgggagtctgaagatggctgggttgtttgtcgtcaggagcaggaagatgatggtggcaaggcagaaggcccaggtgcctggtggcacgcccaccactgacatgatgttggagatggctgcttccatgtatgcacagaacagggcacagatgagggccagcaggtgagtctgccaggtgagggcatagaacatgcctccgatggcgatgcaggagaggacgcagttgtagctccagaggcctgtgtagatggtctcgaagggtgtggccactgacagggctgctagcagccccacgattgagccaatggctgcatgcaagcagatgagtggcgaggagatgaacagagccaccaggaacacgccgcctgtccagggattgtcacagccatacacctggccgaccccaacagggatggcttgtaacagcaggggcatttccatctctgtccaggtgatattgggcactgaagacacaggctctaccagtgttgtggggaagaagaggttgtagtggcctgtggctgcaaggtacaaggtgactgcaatgttgaagggcagagtgaagaccgggaggtcccacttgctgaagatggaattcaaggcactagaaagaactgggcaggacatggctgtgaaggtcacaggaaacagaagccaccagtagtagtctaacttctccgagaacacggccatcagcagtcccaccagcatcccgttgtacccatggagtcctgaggcaatggcagacctgtcttggcccaaggcgagagctgttaaggtcgagaccactgtccccaggcccccagtgattgtccaccagggattctggatcagcagccctatgaagatgatgaggccgctgagaggattgttgatgaacatcacctgagcggtccctctcaggacccagtctatgaactggagggcaaggtgcttgtctttcagccagatcctgtactccttcatgtcgcccgtgaggtagcccactgctttggagaggcagatgcacctttggcctgctgagtcccgatgggccaccccgtcgtctttccttttactcctttcattgagcttttcgatcttcacaatgtgactgtcttcattggaagaccggagatccttttcttcaggcatttccaggaggggcagagctgggtgagtatccggggatgtcgagggccagctcgggctggtaaactctgcctcgtagagtttgtatctgctggaaagtggctctggcaggagaggactgctgtgggggtcagacattccttcgggtcacagccactcttctatcgatggaagtttccttggtcacagtgttgtcagtggttctataaaggtcttatgaatctctacttagttgaccacaagtagtaagcaagaaacaatcggtcattcaggtcctgttggcacaatgaatggaggtgctccaagccttttccttgtctgtaggtagaggtgcaaatacttcaatgagatatgttcctgttcagaaacacccaggatgaaaactggaaagggtcttactgcataatttctttggccacttcagagaatcacagcttcgcagagggaaagtcctttagctgagcagcttcaaaattcttcagctgtgatccacaataagaaacaccttttacattgtgacctgaagaagtctgaaagcaagacgaagagagtccttttgcaagagtgatgtacaaagccctacggacatacagacttcgtgtgcaagtccttaagagaaaattgcaagaaatgagaaagataaagcttgatgaggatgacactatcatgaatcacacgaaaagaaaagaggattatttagcatattgaatatgaagttgtagattcagggcaacatcaagacggatgaactcccccaccaagctgtttaacaaactggctctctgtcgagctggccatgccgagttagtagcagatctgcaatgatgcctctaccaagctcacaattatacaaat

SEQ ID NO: 11369 - RNA, 3585 nt, Homo sapiens
  source 1..3585: mol_type = other RNA
ctgaatagctgggactacaggtgcccgccaccatgcctggctaatttttttttatttttagtagagacagggtttcaccatcttggccaggctaatctcaaactcctgacctcgtgatccacctgcctcggcctctcgaagtgctaggattacatacatgagccaccacgcctggccagctctgtcaaacattaatttgatcccaagcagagggacttttgatctcaatctgcatgagtctgtctctaggaaggaggctgatcattatgctgggggggtgatgagcaccctcccatcttcctctgtccagatctcaggggagagccagcagataggaccattcagcagccaatgtccaaataaggttttgttactcgaagcgctgccaacctactgtgggtcattttattcaggtccatcccaaataaccagaggactcggagtttgcagccaggatggctcagccgcttgcaaagcagtcggacacctgtgtcccctagggcgttgttggtcaggtaaaggtcggtcaaggtctggttgatccccagggtgaagtaaagattctcacaagccttggctgtgaggccacagctatccagccgcagggtctggagcttgcacgtgggatgcctgaggccctcacacagcagcagcaccccgaggtcccccagctcattcaggctcaggtccagctctctcaggctctggttcacactgagagttgaggccagctcgtcacaggcagcagcagtgaggcggcagatcttcagccacaaagtccgtagtctgcagactgggtgcctcagtccctggcatagtaacctcaggcccaaatcctccagtgcatttcctgtcaggtccaactcaaccagatgtgggttggtgccgagcacagaagccatctcctgacaagccccggactccagctgacacttcctcaactgaatcatctgcagcctgcattggggatgccgcaggccctcgcaaagcagcatcatgcctgggaatccaacgccgttgccactgagatccatccttgtcaaattcttattggctatgagagctgcagagaggtcctcgcaggctgagctggagatgcggcacctcttcagcctcaggttctgaagtttgcagttggggtgtctgagtccttgacagagcagcttcaccccccggctgcccagggcatttcggtacagagacagctctatcaggtttggattggtgcacagggccgctgccagatgttcactgtaggcgtccagcagaacggtcctctctggtagctgcaccaacagcgtgtgcgctcctgcggagcacctcgcgcggtcttccccgtccgcgctgtaggtggcgccatacaagtgcagcacctgggcgctcctgcagcgcttcagacagaacgaggagaccatgtgctccatcttggaggcaatgttgctgaccacgatcacctggaagtggctcagggcctgctggataaactcctcctcctggatctcgtacaagcagctgaagaactccaaggagccctgctgcagggtggagccgtcgctctgagctttgctttggatccactgcaacaggtccatcttgatgtgcggcgagaccttccagcagagactcttctccaggtggctcctggtctcctcgttcaggagtccaaacaggaagcggctggtgagtgccaggaagctcctttcagaaaacgcgtactcggtcaacagcctggtcacgtcctggtctgggcctgccccgccctccccctcgtccaggatatagtacatagctgcaaagaattcctggaaactcaagtggatgaagctgtagtacctctcacagttgatgtccttctggaagatgttcatgttgaggaaggcagagacgtcttccccgtctaggccgtgcttccggaggtcctgctcctcaaataggattttctgattccagagcccatctgccgccaaggagcacaaccctctctggttgggtgggggctggaggcgcggggcccccggcttgggttgcatcagactcagcaggtagagcatgtacactgcagtggtggtcctggacgtctgtctcaacagccccccaccctccagctgctgctggaggcaggtacacaccacccagcacaccagggggacgaagcacatggtgaagagaggctcgttgtccctcacgtaattgaagacttggcccgcctgctctgcattgtggaaatacttgtagaagtattccttcctttctgcctcagagaagcccaggatctccacatgcctggggtgctccagcagacggtggagcttctccaaagccgtgggccgtgtggtgatgagcaaagatagctcagggagcagcttcttccgaattaagctgttaagaagcagctccgtgggccgtttctcctcccagcagaggcaccagggtccctgaggatcgtggaaagaaggcttgagctcatcgaagccgtcgatgatgaaaaggaggcgctcgggaactcggatgagctcctggagaggcgcgctgggctcaggccagcagctgaagatgaggtcttgcatgctgcattccgtggcactctggttcatctccctgcagttgatgtagaagagataatcaaatctgccttggaagagcttcccgtccgcccagtccagcatcaccttgtgtgccagcatggacttgcctatccctgccgcgccttgcatgaccacggtgcgcggtggctcggggcgctcctcgtctggctcaaagagggtctctatcttgatggggctagcctggtgtcccacggtcctcgcgtgtccccggcctgtgtccagaagctgctgctggacctgcatggggtttgagtgctccttcaccagcaggagccgggtgtaccggtggctgaggttgacacattcccctaggcgcgcattgcggtcttccatgagccggaatttcctgcggacatagtccctgtaggtttcctggggatcttttcttggagtgacaagagagacttccagaaggcatgttgactggttcccaagtgaggacgggccaccaggtggggtatccctcaccaggtcctctctctgtcctctctcccacaggtccttcctgtttatccgctcaaaggtgctgagagccaacctccaggcctcctctggcccgaagtgggtgatgagcagctgggccatttccaggggaccggccttctccatgcttccccaggggatcttgccttctcccagctctgtcgcggtccccaggtataacttgaacttcttcagttccacagcctcgagttcttccaagtaggtggacaggcgacagaggccgtccctgcctgcggttcgtagcatgggggtgccgtgagccccaaaggagaggacctggaggctgagatgctcctatgcacgggacacagggcgaccccagcacaccttccattgcatcattcacaggcagcgggcggagaggctgagccagtggttggaggagagagcaagggaggaaagaccttttgctgaaataatgctttctcactcttcagttccctcctgccctgccccactcaccaatggctgttct

SEQ ID NO: 11370 - RNA, 1712 nt, Homo sapiens
  source 1..1712: mol_type = other RNA
ctgaatagctgggactacaggtgcccgccaccatgctcggctaattttttttgtatttttagtagagacagggtttcaccgtgttagccaggatggtctcaatttcctgacctcatgatccgccgtgcccagcccttatttcttaagaatagaaaactgtaggaatttgcatagtagatcacctggtgagacctcagtcctatggtgagaaaaattctctataaaagctatatggtccatgatgtcatccaacaccacataagcatataaaatacatgataaggctctccaggaaaaaatattcacaagaaataatgacttctttcatcagcttaaaagtgggaagaacttatttgattaaaaccctgtttaaaatcgattgtcttgttagacttcccctatccataatgaaatcattacagggttctaatgtcaggtggaaaagtgttgactatggagttgtttagcctctgatcctaggataaaccaagcagttaaataatttccaaaagtacaaacagacattcccctcaagttatccgggcttctacaggtacttttcaagtgacccacaagccctatattttaaacagccacagaagtcagaaccaaattcaggtttccaacaaacactgtaaaatgctattcagcaaaagctgcagttccccgtggcagcttgtcaggtggtcagtcagtctcaattactctgggttcctctgcaattgctgtcatgaccgtgagcctctcacgttctacttggctgacagcccaggtctgaggaagtgagagccaacaatcgcttactcagcagcgcattgtgtcgcttcaggtattcaatggtgtctccttgcttttcaacaatttcttctaggcttgaaatagttctaaatcttacctgaatccagtctccgaggtaatattgctggggtaagcatagattttttcttcttcaagtatatcaggctctggtttagctttattaaatctccggattttcactgtgtaaatgaggagacatatcagggaacagatgagttccagtgccaagatggccagaatgaggtcaagatacaatctgccaggctctgggaaggagtgctgcatgcacagtatgaggagaagcactgtgttgccagaggactgtatcatcaacgcaagtctcttgagatgccttgttgatcggtagatcaagttatagcctcggtttctgattttgctgtggtgatactggatgtagcattcaaggagtaaatggagaatccacaaaataactttcccaaggattataaccgtctgaactttcaatgggtttgtgtaatttcctgggcacttgtcctcatttggattaggataagaacaaagcacacctgttaaaaatgctaaaacaacaaacacgagatgaataaaccacagaagattcactatgatgactgtaggaagaggatggaatcggggtctaaagtgagcttgtaatgagtggtgtgggagaagctgggcatccagaagtgggtcgtcttcaatactctgggtgatatccaaggaaccgtcctccatcctgccccccgccgccatttcccgacgccggaggccgaagccctggccagcccggcctctccacctggacctgtaagcctctggccgcgaaactcgccaccttctgggacctgccaggcccctccccagacacaccccctcctgcgtccgccccgcct

SEQ ID NO: 11371 - RNA, 1535 nt, Homo sapiens
  source 1..1535: mol_type = other RNA
ctgaatagctgggactacaggtgcccgccaccatgctcggctaattttttttgtatttttagtagagacagggtttcaccgtgttagccaggatggtctcaatttcctgacctcatgatccgccgtgcccagcccttatttcttaagaatagaaaactgtaggaatttgcatagtagatcacctggtgagacctcagtcctatggtgagaaaaattctctataaaagctatatggtccatgatgtcatccaacaccacataagcatataaaatacatgataaggctctccaggaaaaaatattcacaagaaataatgacttctttcatcagcttaaaagtgggaagaacttatttgattaaaaccctgtttaaaatcgattgtcttgttagacttcccctatccataatgaaatcattacagggttctaatgtcaggtggaaaagtgttgactatggagttgtttagcctctgatcctaggataaaccaagcagttaaataatttccaaaagtacaaacagacattcccctcaagttatccgggcttctacaggtacttttcaagtgacccacaagccctatattttaaacagccacagaagtcagaaccaaattcaggtttccaacaaacactgtaaaatgctattcagcaaaagctgcagttccccgtggcagcttgtcaggtggtcagtcagtctcaattactctgggttcctctgcaattgctgtcatgaccgtgagcctctcacgttctacttggctgacagcccaggtctgaggaagtgagagccaacaatcgcttactcagcagcgcattgtgtcgcttcaggtattcaatggtgtctccttgcttttcaacaatttcttctaggcttgaaatagttctgaatccagtctccgaggtaatattgctggggtaagcatagattttttcttcttcaagtatatcaggctctggtttagctttattaaatctccggattttcacagaggactgtatcatcaacgcaagtctcttgagatgccttgttgatcggtagatcaagttatagcctcggtttctgattttgctgtggtgatactggatgtagcattcaaggagtaaatggagaatccacaaaataactttcccaaggattataaccgtctgaactttcaatgggtttgtgtaatttcctgggcacttgtcctcatttggattaggataagaacaaagcacacctgttaaaaatgctaaaacaacaaacacgagatgaataaaccacagaagattcactatgatgactgtaggaagaggatggaatcggggtctaaagtgagcttgtaatgagtggtgtgggagaagctgggcatccagaagtgggtcgtcttcaatactctgggtgatatccaaggaaccgtcctccatcctgccccccgccgccatttcccgacgccggaggccgaagccctggccagcccggcctctccacctggacctgtaagcctctggccgcgaaactcgccaccttctgggacctgccaggcccctcccc

SEQ ID NO: 11372 - RNA, 1648 nt, Homo sapiens
  source 1..1648: mol_type = other RNA
ctgaatagctgggactacaggtgcccgccaccatgctcggctaattttttttgtatttttagtagagacagggtttcaccgtgttagccaggatggtctcaatttcctgacctcatgatccgccgtgcccagcccttatttcttaagaatagaaaactgtaggaatttgcatagtagatcacctggtgagacctcagtcctatggtgagaaaaattctctataaaagctatatggtccatgatgtcatccaacaccacataagcatataaaatacatgataaggctctccaggaaaaaatattcacaagaaataatgacttctttcatcagcttaaaagtgggaagaacttatttgattaaaaccctgtttaaaatcgattgtcttgttagacttcccctatccataatgaaatcattacagggttctaatgtcaggtggaaaagtgttgactatggagttgtttagcctctgatcctaggataaaccaagcagttaaataatttccaaaagtacaaacagacattcccctcaagttatccgggcttctacaggtacttttcaagtgacccacaagccctatattttaaacagccacagaagtcagaaccaaattcaggtttccaacaaacactgtaaaatgctattcagcaaaagctgcagttccccgtggcagcttgtcaggtggtcagtcagtctcaattactctgggttcctctgcaattgctgtcatgaccgtgagcctctcacgttctacttggctgacagcccaggtctgaggaagtgagagccaacaatcgcttactcagcagcgcattgtgtcgcttcaggtattcaatggtgtctccttgcttttcaacaatttcttctaggcttgaaatagttctgaatccagtctccgaggtaatattgctggggtaagcatagattttttcttcttcaagtatatcaggctctggtttagctttattaaatctccggattttcactgtgtaaatgaggagacatatcagggaacagatgagttccagtgccaagatggccagaatgaggtcaagatacaatctgccaggctctgggaaggagtgctgcatgcacagtatgaggagaagcactgtgttgccagaggactgtatcatcaacgcaagtctcttgagatgccttgttgatcggtagatcaagttatagcctcggtttctgattttgctgtggtgatactggatgtagcattcaaggagtaaatggagaatccacaaaataactttcccaaggattataaccgtctgaactttcaatgggtttgtgtaatttcctgggcacttgtcctcatttggattaggataagaacaaagcacacctgttaaaaatgctaaaacaacaaacacgagatgaataaaccacagaagattcactatgatgactgtaggaagaggatggaatcggggtctaaagtgagcttgtaatgagtggtgtgggagaagctgggcatccagaagtgggtcgtcttcaatactctgggtgatatccaaggaaccgtcctccatcctgccccccgccgccatttcccgacgccggaggccgaagccctggccagcccggcctctccacctggacctgtaagcctctggccgcgaaactcgccaccttct

SEQ ID NO: 11373 - RNA, 3525 nt, Homo sapiens
  source 1..3525: mol_type = other RNA
ctgaatagctgggactacaggtgcccgccaccgcacccggctaatttttttgtatttttagtagagacggggtttcaccgtgttagccaggatggtctggatctcctgacctcgtaatttgcccacctcggcctcccaaagtgctggggttacaggcatgagccaccgcgcccggccttttctgcctttttctattgtggttctctttccctgagactctgttgttctgtctccaactctgggtgtctgacgctgccctctgggtctctgtccctccctcccccactggctctttttgtttgtttgttgagacgggggctccctctgttgcccaggctggagtgcagtggtgcaatcatggctcaatgcagcctctacctctcagggtcaagggatctttctgcctcagcttcctgagtagctgggatcacaggcatgtgccaccacactcagctaatttttgtattttttgtagagatggggtctcaccatgttgcccaggctggtcttgaactcctggcctcaatcaatcccccttcctcggtctcccagagtgctgagattacaggcatgggccacttcgcccggcttctatcccctgctcttggtctctgtctccccactctggatttctgttcctctcttctgcgtctctgccataccccaccctccaggtcattgtctccctctccctgagtctctgtttctctccctttgggtctctgtctctctgggtttccacctcttcctttttctgggtctctttctctatccttttggctctgtccctctatcatgtctggacagagtacagttttctccccctctcccctttcccttgtggctctgacctccatgtctgagcataaaactgtaggggagaatgggagtgaacagcacaatgaagtggatgtggggtaaacaggaggagcatccacctcttcctaatttacccagtcgcctctggatgaacacccaatcccatggatacagaatccagtcccgccccctacagcgagctggggagccagctcggcacacctcccagagccctcgccactgcatgctcccagatacatgatgcttccccactgctatttcctttgggtcctggtgctaccactaaatgcaaaacagcccgatgtggccctatggaactcgttcgcacagtccaactcaacccaacttcctgtaggactcacatagtgacacaactcaatggaactcaattcagcatggccctatgagactcaaacagtggcatgacccaactgaactggccttacaaggctcatatggttgtacaattcaacacaactcaactcgctgtggccacgaaaaatgtccagccacacacctctacacagttaagcccaacagaaccctacaagattcatttggtcatacaaacttaacccaatgtgacctagaaagctcaaattctaccactggactcttcacatttctacatgactcgcaagttcacagaacctaaaataacatgcccctggaagaatcacagagctacacaatttccaccatgtctcaacgaaacttaacaccacacacattcgatctcaacaatgccatgggggaccatctaacttgacccaacatggccctaggggacccaccaaaccacagaatcctacacaatgcagctggaccacactatcccagactcacaacccaaccaaacccaacactgacctaggaaactcacaaaatgatacgaccaaacctatctcaacactaccccaaaaggctccatgagctttgcacaactcagagtaatatgaaccaattgagtcttcattaacacaacacaacccattgccattcgctgctgcttcaggaggtacccacaggagctaccaaaccacacaacccaagacccaacaagactcagtgtttccccactcgttacgacttaacctagctcttcctaaacccaatcccctccccccagccttgccctccaccctgccctccctccctccctctagggaggtgtgaggtcctgcagacctcaactgttcctcacacttcggtgaccaggtgtttccctgggggtgcccagagtggaggtggtagctcaggtacctccccgtccaccagccccccattggccttgccctccagtgggccacaaggctgcatgtccacatggctgaacatcccagcctcttcgccctctgtctcccggtgataaaagtagctgaaattggagacaatgacgggcactggcagggaaatagtcagcacgcccgcaatggcacacagagagcccactatcttgccacccacagtgacgggtgccatgtctccatagccaactgtagtcatggtgactaccgcccaccagaaggactcagggatgctagtgaaatgggagtccacccggtcaacttcggcaaagtagacggcgctggaaaagaggaccacaccgatgaagaggaaaaagatgaggaggcccagctcacgcatggaggcccgaagcgtctggcccaagatttgcaggccctttgagtgccgggacagcttgaagatgcggaagacacgcaccaatcggatgactctcaggatggccagtgacatggcctgctggcccacccctcgctgccgggccagctcggtgcccagtgccacaaagtagggaaggatagccacaaaatcgatgaggttcatcacgttcttgaagaagatagccttgcttggacagaccaggaggcgtaccagcagctcaaaggagaaccaacaaatacacagcgtctccaccacgaagaacgggtcattgaagggcaggcggggtggatttccaggcatttggctggagccattcagcggagcggggaacgggccggctgcggctgcagcagcaagccccgtgccgtcgcggtcgtcgcggaagtcaggcagcgtctcgaggcagaagacgacgatggagacgaggatgaccagcacggagactacggcgagcacgcgcgcggcctgagagctctcgggaaactcgaaaagcagccacagctggcgggcgaaggcgcggcggggcagggggcgctcgggcggcaccgggcagccctcgtcctcgcgcaggcgtgccagggccgccgcgcccagcccgtagaaggccacctcttccaggaagacgtcgagcggcacgtgcgccggccgccgcagccgcccaccggactggtagtagtagagcacggcgtcgaagctgggccggtgccggtcgaagaaatactcgcggcgcgcgtcgtcgtagaagcggccgcggcgcgctgggtcccctagcagagtgtccgggaagcggcccagcgtgcgcgcccgcgtctcgaagcgcagcccggccacgttgagcaccagccgctcgcagcagccgcacggcggcgggcaccgcggctccatggcgcgcgcagccccggcgacccgcgaaccgacgtgtggccccgacgcccggccccggtgcggccccgcctcggccgcctcggccgccgccgccgccgccccagcccggtgtcc

SEQ ID NO: 11374 - RNA, 1438 nt, Homo sapiens
  source 1..1438: mol_type = other RNA
ctgaatagctgggactacaggtgcccgccaccgcgcccggctaaattttttttgtatttttagtagagacggggtttcaccatgttagccaggatggtctcgatctcctgacctcgtgatccacccgcctcggcctcccaaagtgctgggattacaggcgtgagccaccgcgcccggccccctcctccccaatttttcatacagttgcccctatacaatatacacacccttgagggcaggtagaagtccagcccacctgcgccagggacgctgtggggagcatttttctctgagttgctaagagaaccctgatgggcggtgagcagaggaaccacagaacagccagggctcaaggctggcagcggataggccaggagagatcgctaggccccagaaagccccctactttcagtcaggatgggcaagagggtcttcgcagtgaagtgggaggcaggcctggaggagggagccagggagacccctgggagccctgaggttgggggccaggcagggagatggggatagcagctgcctcagtacttggggaccttgctgtagtcttcggaatggacgtgccggcacaagcagatggacaggaccatccccaggagctcgatgatggccacacccacgcccacgccgaggatgatgcccaggttctcctgcagccacgcctgcaccttctccatgcagccctcctggtacacaggccagtcctcagggtggttgccactctgggtcctgttgccgggggcctcgcagaagcccttcctcacagaaaggctgttgtcctcttcccccttgacttcgcaggaacaggggtaggtgacctcagggcgattcatgagctcagcgttgtctgtccagttgtagaagctgacccagccgcagcacttcacctgagcctgcacgtagtcccaggcatcctgcaggctgtcctcgcgactgctgttgtagtctcgaatgagctcagtcacgatgccgcccatctcctgcttcagcagccccagcaggcagcggacctcgttgacggcgccgatgcagcccaggaagcccatgagcatagtgactgcccccacgccgatgaagacataggcccccatcctaagcgagctggaggaggtttgcaggacagagatgaaactgctcttgtcggccaggatccacaccccgaagcccaggatcactgcgcccaggataaagaagatcaagttgaagaggaagagaaagtatttggtgactttgatacaggctgagcccatcccgccagtcctggagcttccttccacgaaaccagtgcagctggtcacagggcccacttctgcctgtgcccacgtgtcgtccacacagcagcagggaggactctgcgggttctgctttctgctccgcgctgcaggcccagcgtcacccgctcgtgcctcagtcggcgtcggactgc

SEQ ID NO: 11375 - RNA, 1513 nt, Homo sapiens
  source 1..1513: mol_type = other RNA
ctgaatagctgggactacaggtgcccgccaccgcgcccggctaaattttttttgtatttttagtagagacggggtttcaccatgttagccaggatggtctcgatctcctgacctcgtgatccacccgcctcggcctcccaaagtgctgggattacaggcgtgagccaccgcgcccggccccctcctccccaatttttcatacagttgcccctatacaatatacacacccttgagggcaggtagaagtccagcccacctgcgccagggacgctgtggggagcatttttctctgagttgctaagagaaccctgatgggcggtgagcagaggaaccacagaacagccagggctcaaggctggcagcggataggccaggagagatcgctaggccccagaaagccccctactttcagtcaggatgggcaagagggtcttcgcagtgaagtgggaggcaggcctggaggagggagccagggagacccctgggagccctgaggttgggggccaggcagggagatggggatagcagctgcctcagtacttggggaccttgctgtagtcttcggaatggacgtgccggcacaagcagatggacaggaccatccccaggagctcgatgatggccacacccacgcccacgccgaggatgatgcccaggttctcctgcagccacgcctgcaccttctccatgcagccctcctggtacacaggccagtcctcagggtggttgccactctgggtcctgttgccgggggcctcgcagaagcccttcctcacagaaaggctgttgtcctcttcccccttgacttcgcaggaacaggggtaggtgacctcagggcgattcatgagctcagcgttgtctgtccagttgtagaagctgacccagccgcagcacttcacctgagcctgcacgtagtcccaggcatcctgcaggctgtcctcgcgactgctgttgtagtctcgaatgagctcagtcacgatgccgcccatctcctgcttcagcttgcccatgttgaagtagaagagggccccggccgtcacctgggcaatgaggatcaggagcaggaaagcaaagtacagccccagcaggcagcggacctcgttgacggcgccgatgcagcccaggaagcccatgagcatagtgactgcccccacgccgatgaagacataggcccccatcctaagcgagctggaggaggtttgcaggacagagatgaaactgctcttgtcggccaggatccacaccccgaagcccaggatcactgcgcccaggataaagaagatcaagttgaagaggaagagaaagtatttggtgactttgatacaggctgagcccatcccgccagtcctggagcttccttccacgaaaccagtgcagctggtcacagggcccacttctgcctgtgcccacgtgtcgtccacacagcagcagggaggactctgcgggttctgctttctgctccgcgctgcaggcccagcgtcacccgctcgtgcctcagtcggcgtcggactgc

SEQ ID NO: 11376 - RNA, 1624 nt, Homo sapiens
  source 1..1624: mol_type = other RNA
ctgaatagctgggactacaggtgcccgccaccgcgcccggctaaattttttttgtatttttagtagagacggggtttcaccatgttagccaggatggtctcgatctcctgacctcgtgatccacccgcctcggcctcccaaagtgctgggattacaggcgtgagccaccgcgcccggccccctcctccccaatttttcatacagttgcccctatacaatatacacacccttgagggcaggtagaagtccagcccacctgcgccagggacgctgtggggagcatttttctctgagttgctaagagaaccctgatgggcggtgagcagaggaaccacagaacagccagggctcaaggctggcagcggataggccaggagagatcgctaggccccagaaagccccctactttcagtcaggatgggcaagagggtcttcgcagtgaagtgggaggcaggcctggaggagggagccagggagacccctgggagccctgaggttgggggccaggcagggagatggggatagcagctgcctcagtacttggggaccttgctgtagtcttcggaatggacgtgccggcacaagcagatggacaggaccatccccaggagctcgatgatggccacacccacgcccacgccgaggatgatgcccaggttctcctgcagccacgcctgcaccttctccatgcagccctcctggtacacaggccagtcctcagggtggttgccactctgggtcctgttgccgggggcctcgcagaagcccttcctcacagaaaggctgttgtcctcttcccccttgacttcgcaggaacaggggtaggtgacctcagggcgattcatgagctcagcgttgtctgtccagttgtagaagctgacccagccgcagcacttcacctgagcctgcacgtagtcccaggcatcctgcaggctgtcctcgcgactgctgttgtagtctcgaatgagctcagtcacgatgccgcccatctcctgcttcagcttgcccatgttgaagtagaagagggccccggccgtcacctgggcaatgaggatcaggagcaggaaagcaaagtacagccccagcaggcagcggacctcgttgacggcgccgatgcagcccaggaagcccatgagcatagtgactgcccccacgccgatgaagacataggcccccatcctaagcgagctggaggaggtttgcaggacagagatgaaactgctcttgtcggccaggatccacaccccgaagcccaggatcactgcgcccaggataaagaagatcaagttgaagaggaagagaaagtatttggtgactttgatacaggctgagcccatcccgccagtcctggagcttccttccacgaaaccagtgcagctggtcacagggcccacttctgcctgtgcccacgtgtcgtccacacagcagcagggaggactctggaaaagccccactgagtttccaacttgaagtcttagggggtccggctcagttgaactgcgggttctgctttctgctccgcgctgcaggcccagcgtcacccgctcgtgcctcagtcggcgtcggactgcacagcccggggctcagtcactcctcggccccctcccggctgcagccggggaac

SEQ ID NO: 11377 - RNA, 1287 nt, Homo sapiens
  source 1..1287: mol_type = other RNA
ctgaatagctgggactacaggtgcccgccaccgcgcccggctaaattttttttgtatttttagtagagacggggtttcaccatgttagccaggatggtctcgatctcctgacctcgtgatccacccgcctcggcctcccaaagtgctgggattacaggcgtgagccaccgcgcccggccccctcctccccaatttttcatacagttgcccctatacaatatacacacccttgagggcaggtagaagtccagcccacctgcgccagggacgctgtggggagcatttttctctgagttgctaagagaaccctgatgggcggtgagcagaggaaccacagaacagccagggctcaaggctggcagcggataggccaggagagatcgctaggccccagaaagccccctactttcagtcaggatgggcaagagggtcttcgcagtgaagtgggaggcaggcctggaggagggagccagggagacccctgggagccctgaggttgggggccaggcagggagatggggatagcagctgcctcagtacttggggaccttgctgtagtcttcggaatggacgtgccggcacaagcagatggacaggaccatccccaggagctcgatgatggccacacccacgcccacgccgaggatgatgcccaggttctcctgcagccacgcctgcaccttctccatgcagccctcctggtacacaggccagtcctcagggtggttgccactctgggtcctgttgccgggggcctcgcagaagcccttcctcacagaaaggctgttgtcctcttcccccttgacttcgcaggaacaggggtaggtgacctcagggcgattcatgagctcagcgttgtctgtccagttgtagaagctgacccagccgcagcacttcacctgagcctgcacgtagtcccaggcatcctgcaggctgtcctcgcgactgctgttgtagtctcgaatgagctcagtcacgatgccgcccatctcctgcttcagcttgcccatgttgaagtagaagagggccccggccgtcacctgggcaatgaggatcaggagcaggaaagcaaagtacagccccagcaggcagcggacctcgttgacggcgccgatgcagcccaggaagcccatgagcatagtgactgcccccacgccgatgaagacataggcccccatcctaagcgagctggaggaggttttgtgcctcatgggctttccacacgccgtctccaactctgacatcaccctgcctggcaggcactagcatggccatttcacagaagaa

SEQ ID NO: 11378 - RNA, 1686 nt, Homo sapiens
  source 1..1686: mol_type = other RNA
ctgaatagctgggactacaggtgcccgccaccgcgcccggctaattttttgtatttttagtagagacggggtttcaccgtgttagccaagatggtctcgatctcctgaccttgtgatccgcccgcctcggcctcccaaagtgctgggattacaggcgtgagccaccgcgcccagccgacagaatatatcttatgcatttttatttattgaatgtcattttattccaatgataagatacagattacaaaacttctagtataattacacataattaccttttgttgttttcctacaagaaatgcacaggtattttgaggtcttttgtattgcattattggtaaaacattgcatagtattagtttgtggctctgttacaatgggtaatgacaggaatgcatacagatgtctctgctatgataaaatgtgctcttgttgggttacattaaccttccttcaaaagggatttctcagttgtacttcttacagtcttcaggaaattcattaaatcagtgcctccagttcctttggcttccagttttgaagggtcttcagaggtcttattctcctttggctgctggcttgcaggaatcaggatgtacttagtcacgatttgcagatggtagctcctcagggagaccagagctttcacacaggcgtcataagcttcccgcaggccagcatcaccttttgaaaggacaaactcacggactgagggatttgactctaatgagcacaggaagttcctgtgagctggtggcatatatcttctcatgtcctggaggaactgagcagcatgtcctccaccagcagtctgctggatgcccagcaggacgtcaaagcactgaaagacgctgctttggcctgcactgccccctgcaaactcctttgggtcttcccagaacccttcatacaccagaccgtctgatagctgggggttgcctttccagccagacaaatatatgcgaagaacactgaaaaatgcttttgggttcacatgatcgtggatttggtgaaacacttgaagggctttctccaagcaagaagctatttccaacagcgcctttagcaaagtgtcccgttcttgcatttgcattgccttgaatacagtaggaattactttgattgcagaagcagctgctatttccaccaatagagagaccaggaagaatcctttactgcagtctccatcacgaaatgagaacaaaacgtccatgttctcataagtcaggggcttattaggatcctttttcttccagtttgccaagacacagtctgcataaaccaaaataggaggcagttccagtttcttggagagttggcagtaaggaacagcaatatttcttggcaagaccttacggacatctccatgacctttgccccacacatatgccatggtgatgcatcccagaactagacgtgcaaggcgctgtgacttgtggtctgtgagatgatcaatgctgagcatgtttaacttctcaactctttctcgaagctggccagactctatgagatcaggcagatgtttagcaatgaacatccagtcattataaaaatcaggtagattttcctgtggatttggcagagcaaagcccacttcttcatcaatatggtactctttactgattgtccaggagttttccatagcgtgtgccattcttgtagtctgctcctctggtgcccctcagt

SEQ ID NO: 11379 - RNA, 3351 nt, Homo sapiens
  source 1..3351: mol_type = other RNA
ctgaatagctgggactacaggtgcccgccacctcgcccagctaattttttgtaattttagtagagatggggtttcaccatgttagccaggatggtctcgatctcctgacctcatgatccgcccacctcggcctcccaaagtgctgggattacaggtgtgagccaccgcgcccagctaagaattgtttttatgaaattattgagagattttgcctcctgcttcctttctggtattgagaggtaagtagttgatcactttatcccgtttgctttggctttaaagacggtcaaggataaattcaatagagccatgataaccatgctggccaaataaatctgtgcagatttttcccatacaactttctggctttatttctcctggtttgaattttttagactatggttttattatatatatattatatatgcttggagctgcatcaagggtcagtgagatttacttcacaggaggaaaccaaggggagcagagggaagtaggaagcccggcttggtatggctacaatggctaggtgatagagtactttggacgaatggctcttgagacgaatggctcttggttcagggaacggcacagtgggggcgtggctgaagcagtatactcggaaatctgctctgaggaaccagagcaaactgtacagaggaaaggggagaatggaggccagtgattggctgtgaggtgctgccataacccaggtaggagagacccacaggctagcagctgctttgagaacacaggacacattcatgagaatctctgtctcctaacttgattcaacacaaattaagatatttcacttacacaggtatgcttgtttcttaaaacaattaatttgaaaaataagaggtttttaacctactctatttgacttctgagtccctcaaatctctgcggtgtcttttaagtttacaagtgagatgggtactgcctcagaaatataacaattatttttttccttatatataaactttatatataaaatctatactttataagtatcaaactattatacatgaggtaatattaggaagtaaactgctagactgtagtataagattaactacaagtattgacaaggctcatgaaaattaaaaaattaagcattcctatttattccctttctatgcaatgaattgcattatccactgtataaggttgttatgagacttaaataagaagtgccttgcccacctcccgagccacagctgagaagcgaaccaatcaacctgggcagacagcaaaagggcactgagagatgacttgctctccattcctcagtttcctgcttctaagggcctaggatttacccttgtttcctgctttctttcgtcttgtctgataaacctttgcttggagtatatgcaattccctttcttgctttagcaggattagataacaatgaaaataactttgattcctattttcaaataggactttgctaagaagtatcactagctttggtgtactctgtatgtccagcaagttggtaatactattacttttcccaacaataaaacaatataatgacgagtttccatttcatggtatttgtctaataataaccaataatcaatattactatataaaactgcatatttagaatctcattattatttgtacttggaacattagtatttgaatcttgtgttaatgataccatcacactcctaaagtttgtaactcacacaagtgtataatctgactacagtttataaaccaatgagaaagataaatattcttatattttaacaacagaaaagttacgaactctaaatttagaaatggtatagtaagagatattgtttcactttatttataatagtaagaaactggaaacaaatgtctaacaataggaaactggtttaaaaaaatcatagaaccataatttattttaagccctaaaatgaaattgtgaaccattaaaaatatgttgtaaaactatttaatgtcataaagagaactaactctgtttttatggtccatctaccaatgtcttccgagcagttctctctcctcaaacctcctctacctctttactcaccctcactcagcctaaccttgcttccgattttattaaggaaatccaatcaatcagaagaggtttctacaatttactatcacatttacccaccagccatcacctctgccatatatgctcctctcctattccaatggctggaatgtctcagggaagaccaagcccttcacttgtacattagatcccagctctctgtcccatccattatggaagctgcacatcaccccagtcacacaagagggcactctgaatgaggaatcttgtaaactactccaaatcaccagtcttgaacagtcttgaacacgcatgggcgttaaagtactctttatctgtacattgctacctttttatgtctattttatttacatgacttcttttcagtatccaaaactttagccaacaattcttgtgtttcaggagtcagtggagcatgagaaaacttgcagtattctccctgataacattttgttcctgtatggtaaaacttacaaggatattcattatgcaaatacagacagttttcacctctggtacaatatccttgtacataaaacttacacatttcctttttcttttctatctctgcatcatgatcaaatttacactggtctcccttaatacatttcctttcaagaaaatatttacaaatttgttttcccttgcgttccactgtatgttggttgatgaatgcctgactcaaatgctgctgcttctctttaggtttaccatcctcttcctgtgagccgctgttcctcagcaaagcatttgatcctttgtttccagggccaggccattttcgcttcattttcttctgtttgccattcttgtgaccagctttaagatttttatttttttgtttagcagcctgtggggtatcttttactccttctttctttgtagattcttcaggttgagcagcatttgccatttctctggcttgtatgtactgttgaagctctttggcaaaattatcttctgattcctgactgcagatatcattatcactatatacatcatagtccttacttcttgattttctatgcagcgaactttttggtgatattgcagagtgtctaaattttttgggaatttgctcgcactccagtttaattttctcttcttgtgtttcttcaacttctgtatctatttcatcatcgattctttcgtcagagtccgtggccgttttgccgagggccgggttggggggttttgagaaaagattctcaaaatccatgacccagacaggtcctccctttcgcgagccgggaagctacagagtaacaacccgagagagt

SEQ ID NO: 11380 - RNA, 2238 nt, Homo sapiens
  source 1..2238: mol_type = other RNA
ctgaatagctgggactacaggtgcccgccactacgcccggctaattttttgtatttttagtagagacggggtttcaccgttttagccgggatggtctcgatctcctgacctcgtgatccgcccgcctcggcctcccaaagtgctgggattacaggcgtgagccaccgcgcccggccacaagtatttcttgtaagcctgctacacatactgttctcggtgatggcagatgtagcagtaaataaaacaagataaaacaaagcccttgttttcacagagcatccattatggtaaggggagaaaaggaaataaaaacatgtcaagaaaaaaaaggacagtaattttatataaaataaagacattcatctttgtgttaaagatagatatactgagcaaaccttttacttatgctctcatttaattggtatcttgaaaggtaccaactgcctcccaatcaccaaattaaacagaattttctcagtctccattttccttatattcctctaagcatctgatactgctcaccaccttcattttgaaactccaatggtttgcatgacaaatttcctattctggttcttatcttttcacattagtgtgacattaacataagctacacggtcacatctaggatttgagaccattccctatccaacaaaaggaaacggatttaattgatgtagaaatcggacagcacctagagaaaagttttcactttgttcttaatttccaataggttttagaatattattatcaatgtaattacatttattcaacgcactagagagtaacaacatcaataagcacctgtacaaaatgttacattttataaaaccctttcacatttacttcatttaatcctcataaaatgaaaataaccccataatagttgcacattaaaaacaaagtcctgcttttcagaatgacttcactaaaaaactagacttaaatagtatcctttatttttcctttaatatttggaaactaccttaaagtataatgaaaaaacataagaaacatctgtaatcccaatattcaaaaataacatttgctaacattttgctacattgaacatttcttccatcccatccctattaactttaataatttttaattgcttcatactaactagaatattaatattctgtaaaaaagaagtctgttttttatttaaaaataaacaatccaggtgggggaccatactgatcaaactgactgtgaagtcaactcaaacaatttttataattttttaagttgtagttttagagttacaggtggaaaaagaaatgaagcatatttattcaataaatgtttacatgtgcaaagcaacacaaacaaaaattatgtacatgaagacaactagactctcacctgttcaatctctttggtttttgatgctattgctttagagcgagtggttagctgactatcttcaaataattctatcccatgtgttgtgtttgactcaggttcctctggctggtcagtaaacaatggtgctgtggatcccgcctcatactcagaaatttcaggcaagttactttcatctgatttctctagcttttcagcagcccacttgcttgcagcctcagcaagttccttttcagttagcctactgggtttgtctaacacctttgatgaagaaactgctgaaccacttgagggtgaagtatctcttgatgttttcaaagactggacaggcctctctttatctctttcaggatttccttcattctgccgtttgtaggaggcaccaggacgcacggactttctatgttgagactgatggaaagagtatgatttgctcctttctggagagtagcttctgctactgacactggaaccagatctgctgtgtggagaatcctttcggccaacaggtgattctctgaaaaaagtattgtcccttttataaggagaccgctctctcgcataatgggaagagtagaaactttttcttctaaagccatctctcatgtccctgtattcaggttgcctgcttgcagaatgatcgtctcttgtccatctataaccagattcatcactgggatgacttcgaggaggtgctcgttctctcggaattctttcatattcatatcgtccctcagaccacatttcgtctcttctgtaagccattgagtccttttaggaatcaaatttaacgttttcaacaatttccgactctggccctccgggagaccccgtaaatgcagccgtccgctcgccgccgttatcccaggt

SEQ ID NO: 11381 - RNA, 2360 nt, Homo sapiens
  source 1..2360: mol_type = other RNA
ctgaatagctgggactacaggtgcccgccactacgcccggctaattttttgtatttttagtagagacggggtttcaccgttttagccgggatggtctcgatctcctgacctcgtgatccgcccgcctcggcctcccaaagtgctgggattacaggcgtgagccaccgcgcccggccacaagtatttcttgtaagcctgctacacatactgttctcggtgatggcagatgtagcagtaaataaaacaagataaaacaaagcccttgttttcacagagcatccattatggtaaggggagaaaaggaaataaaaacatgtcaagaaaaaaaaggacagtaattttatataaaataaagacattcatctttgtgttaaagatagatatactgagcaaaccttttacttatgctctcatttaattggtatcttgaaaggtaccaactgcctcccaatcaccaaattaaacagaattttctcagtctccattttccttatattcctctaagcatctgatactgctcaccaccttcattttgaaactccaatggtttgcatgacaaatttcctattctggttcttatcttttcacattagtgtgacattaacataagctacacggtcacatctaggatttgagaccattccctatccaacaaaaggaaacggatttaattgatgtagaaatcggacagcacctagagaaaagttttcactttgttcttaatttccaataggttttagaatattattatcaatgtaattacatttattcaacgcactagagagtaacaacatcaataagcacctgtacaaaatgttacattttataaaaccctttcacatttacttcatttaatcctcataaaatgaaaataaccccataatagttgcacattaaaaacaaagtcctgcttttcagaatgacttcactaaaaaactagacttaaatagtatcctttatttttcctttaatatttggaaactaccttaaagtataatgaaaaaacataagaaacatctgtaatcccaatattcaaaaataacatttgctaacattttgctacattgaacatttcttccatcccatccctattaactttaataatttttaattgcttcatactaactagaatattaatattctgtaaaaaagaagtctgttttttatttaaaaataaacaatccaggtgggggaccatactgatcaaactgactgtgaagtcaactcaaacaatttttataattttttaagttgtagttttagagttacaggtggaaaaagaaatgaagcatatttattcaataaatgtttacatgtgcaaagcaacacaaacaaaaattatgtacatgaagacaactagactctcacctgttcaatctctttggtttttgatgctattgctttagagcgagtggttagctgactatcttcaaataattctatcccatgtgttgtgtttgactcaggttcctctggctggtcagtaaacaatggtgctgtggatcccgcctcatactcagaaatttcaggcaagttactttcatctgatttctctagcttttcagcagcccacttgcttgcagcctcagcaagttccttttcagttagcctactgggtttgtctaacacctttgatgaagaaactgctgaaccacttgagggtgaagtatctcttgatgttttcaaagactggacaggcctctctttatctctttcaggatttccttcattctgccgtttgtaggaggcaccaggacgcacggactttctatgttgagactgatggaaagagtatgatttgctcctttctggagagtagcttctgctactgacactggaaccagatctgctgtgtggagaatcctttcggccaacaggtgattctctgaaaaaagtattgtcccttttataaggagaccgctctctcgcataatgggaagagtagaaactttttcttctaaagccatctctcatgtccctgtattcaggttgcctgcttgcagaatgatcgtctcttgtccatctataaccagattcatctcctctgtgaggtggaccacttcttcgatcatgagaaaaactgcggccctcgtcatagtctcggtaatcaacatgactgtaatatctattgtagcttccttcaccaggtctgtctagcagtggtggtttctttggcacaatattaactagtctattgtagccatcactgggatgacttcgaggaggtgctcgttctctcggaattctttcatattcatatcgtccctcagaccacatttcgtctcttctgtaagccacgactctggccctccgggagaccccgtaaatgcagccgtccgctcgccgccgttatcccaggt

SEQ ID NO: 11382 - RNA, 2138 nt, Homo sapiens
  source 1..2138: mol_type = other RNA
ctgaatagctgggactacaggtgcccgccactacgcccggctaattttttgtatttttagtagagacggggtttcaccgttttagccgggatggtctcgatctcctgacctcgtgatccgcccgcctcggcctcccaaagtgctgggattacaggcgtgagccaccgcgcccggccacaagtatttcttgtaagcctgctacacatactgttctcggtgatggcagatgtagcagtaaataaaacaagataaaacaaagcccttgttttcacagagcatccattatggtaaggggagaaaaggaaataaaaacatgtcaagaaaaaaaaggacagtaattttatataaaataaagacattcatctttgtgttaaagatagatatactgagcaaaccttttacttatgctctcatttaattggtatcttgaaaggtaccaactgcctcccaatcaccaaattaaacagaattttctcagtctccattttccttatattcctctaagcatctgatactgctcaccaccttcattttgaaactccaatggtttgcatgacaaatttcctattctggttcttatcttttcacattagtgtgacattaacataagctacacggtcacatctaggatttgagaccattccctatccaacaaaaggaaacggatttaattgatgtagaaatcggacagcacctagagaaaagttttcactttgttcttaatttccaataggttttagaatattattatcaatgtaattacatttattcaacgcactagagagtaacaacatcaataagcacctgtacaaaatgttacattttataaaaccctttcacatttacttcatttaatcctcataaaatgaaaataaccccataatagttgcacattaaaaacaaagtcctgcttttcagaatgacttcactaaaaaactagacttaaatagtatcctttatttttcctttaatatttggaaactaccttaaagtataatgaaaaaacataagaaacatctgtaatcccaatattcaaaaataacatttgctaacattttgctacattgaacatttcttccatcccatccctattaactttaataatttttaattgcttcatactaactagaatattaatattctgtaaaaaagaagtctgttttttatttaaaaataaacaatccaggtgggggaccatactgatcaaactgactgtgaagtcaactcaaacaatttttataattttttaagttgtagttttagagttacaggtggaaaaagaaatgaagcatatttattcaataaatgtttacatgtgcaaagcaacacaaacaaaaattatgtacatgaagacaactagactctcacctgttcaatctctttggtttttgatgctattgctttagagcgagtggttagctgactatcttcaaataattctatcccatgtgttgtgtttgactcaggttcctctggctggtcagtaaacaatggtgctgtggatcccgcctcatactcagaaatttcaggcaagttactttcatctgatttctctagcttttcagcagcccacttgcttgcagcctcagcaagttccttttcagttagcctactgggtttgtctaacacctttgatgaagaaactgctgaaccacttgagggtgaagtatctcttgatgttttcaaagactggacaggcctctctttatttctatgttgagactgatggaaagagtatgatttgctcctttctggagagtagcttctgctactgacactggaaccagatctgctgtgtggagaatcctttcggccaacaggtgattctctgaaaaaagtattgtcccttttataaggagaccgctctctcgcataatgggaagagtagaaactttttcttctaaagccatctctcatgtccctgtattcaggttgcctgcttgcagaatgatcgtctcttgtccatctataaccagattcatcactgggatgacttcgaggaggtgctcgttctctcggaattctttcatattcatatcgtccctcagaccacatttcgtctcttctgtaagccacgactctggccctccgggagaccccgtaaatgcagccgtccgctcgccgccgttatcccaggt

SEQ ID NO: 11383 - RNA, 2303 nt, Homo sapiens
  source 1..2303: mol_type = other RNA
ctgaatagctgggactacaggtgcccgccactacgcccggctaattttttgtatttttagtagagacggggtttcaccgttttagccgggatggtctcgatctcctgacctcgtgatccgcccgcctcggcctcccaaagtgctgggattacaggcgtgagccaccgcgcccggccacaagtatttcttgtaagcctgctacacatactgttctcggtgatggcagatgtagcagtaaataaaacaagataaaacaaagcccttgttttcacagagcatccattatggtaaggggagaaaaggaaataaaaacatgtcaagaaaaaaaaggacagtaattttatataaaataaagacattcatctttgtgttaaagatagatatactgagcaaaccttttacttatgctctcatttaattggtatcttgaaaggtaccaactgcctcccaatcaccaaattaaacagaattttctcagtctccattttccttatattcctctaagcatctgatactgctcaccaccttcattttgaaactccaatggtttgcatgacaaatttcctattctggttcttatcttttcacattagtgtgacattaacataagctacacggtcacatctaggatttgagaccattccctatccaacaaaaggaaacggatttaattgatgtagaaatcggacagcacctagagaaaagttttcactttgttcttaatttccaataggttttagaatattattatcaatgtaattacatttattcaacgcactagagagtaacaacatcaataagcacctgtacaaaatgttacattttataaaaccctttcacatttacttcatttaatcctcataaaatgaaaataaccccataatagttgcacattaaaaacaaagtcctgcttttcagaatgacttcactaaaaaactagacttaaatagtatcctttatttttcctttaatatttggaaactaccttaaagtataatgaaaaaacataagaaacatctgtaatcccaatattcaaaaataacatttgctaacattttgctacattgaacatttcttccatcccatccctattaactttaataatttttaattgcttcatactaactagaatattaatattctgtaaaaaagaagtctgttttttatttaaaaataaacaatccaggtgggggaccatactgatcaaactgactgtgaagtcaactcaaacaatttttataattttttaagttgtagttttagagttacaggtggaaaaagaaatgaagcatatttattcaataaatgtttacatgtgcaaagcaacacaaacaaaaattatgtacatgaagacaactagactctcacctgttcaatctctttggtttttgatgctattgctttagagcgagtggttagctgactatcttcaaataattctatcccatgtgttgtgtttgactcaggttcctctggctggtcagtaaacaatggtgctgtggatcccgcctcatactcagaaatttcaggcaagttactttcatctgatttctctagcttttcagcagcccacttgcttgcagcctcagcaagttccttttcagttagcctactgggtttgtctaacacctttgatgaagaaactgctgaaccacttgagggtgaagtatctcttgatgttttcaaagactggacaggcctctctttatttctatgttgagactgatggaaagagtatgatttgctcctttctggagagtagcttctgctactgacactggaaccagatctgctgtgtggagaatcctttcggccaacaggtgattctctgaaaaaagtattgtcccttttataaggagaccgctctctcgcataatgggaagagtagaaactttttcttctaaagccatctctcatgtccctgtattcaggttgcctgcttgcagaatgatcgtctcttgtccatctataaccagattcatctcctctgtgaggtggaccacttcttcgatcatgagaaaaactgcggccctcgtcatagtctcggtaatcaacatgactgtaatatctattgtagcttccttcaccaggtctgtctagcagtggtggtttctttggcacaatattaactagtctattgtagccatcactgggatgacttcgaggaggtgctcgttctctcggaattctttcatattcatatcgtccctcagaccacatttcgtctcttctgtaagccacgactctggccctccgggagaccccgtaaatgcagccgtccgctcgccgccgttatcccaggt

SEQ ID NO: 11384 - RNA, 7229 nt, Homo sapiens
  source 1..7229: mol_type = other RNA
ctgaatagctgggactacaggtgcccgccactatgcctggctaatttttgtatttttagtagagatggggtttcgccatgttggtcaggctggtcttgaactcctgacttcaggtgatccacccacctcggcctcccaaaaggctgggattacaggtgtgagccaccgcacccagccataagttcttttttctaagtacatgctataatgcaattcatgtaatgccactgagatttcctaaagccaacaaacaaaattctaaaattgtactgttaaagaaaacactgaagacttatccttgattcttttccaaagctaacatcaacctaactcatttattgtctcataaatgtctagatacctaccacgcacaaagtcctatctaggtactaggggcatataatctctgtactcaagagatatagactctttcttcttcttttgctttttttttttttttaagagataagatctcgttatattgcccaggctggtctcaaattcctgggctcgagtgaacctcctgagtagttgggactactactcaccacacatggcaataaagattctaaagttagaaggacaaagtgatgttacctaaatttgcctgtgcttctgatatgacaaataatccgccactggtgcatggcccatagagctcatcttcatctttggatgaatacgagtggacctgtcatactcctcagccctatgacatgtaaagcacaaagccaggaatgaggtcattgtcttatcacttacccccaaaagctctcaatggctcaacttacctaagtcttcctcctttattctcttccttcatatcaaaacttctgcaaatttttataataattttttaaatgagtaaactgatctggaaaaaatatttttttcagtttttatttcaataaaacaagaggcaacacttgttgtataaagtactacatatggagaacatttacacaaatatacaaaaattcaaaaaactaaactccagtttatttccatagccttaagaaggtagggaacacacaaaaatagccaaagtcgtcgtttattctttaggaatgtaaactctaggaatacaattagaaacaaatatatttactatgaaaagattagtatcactaaatgattagaaataaaggtaagaggtacacaataagttccatataagagaaagcaacaatacgtgaaataaaatcttgggtttatggtaaaaacttcctattaagacaaatgtactctaaaactctactataaaaaaacacaaaaacatctcccaaaatgttcgttgttagtttctttagatatgcacaagttacaaagtatagaagacaatatatttatgctctctgatgaagaatttaacaatattaaacataaatctgaataactcaaagtactgagtataattttactaagcaacaaatgtagaagtataaattcatgctcattaaaggactagagagttttaatttttcatacaaagactgggaggacactattatacattaatttctatctacaatgcttaaagtacccatcaaattatttttctttttaagtggtttttaaaaaatatttttcagttacattattcaacatgtatatatttccttgatgtgcttccctttaatacagatttattgtgcctaaacgcaaatgttaacctgccttattttaaatatttgtttaaaattatgtctcagagtacatctgttctctgtaattcaacagttttaacattttagttttattcttccaaaataggcaaaatcccttaaaactgggatcattttgatctattttggttttaaaaatatatttccctttaattcaactttttaaaaaaatgagtaatatttgctgagcagttgcttcacaattgaaaagagcaatgaaatattgctttttcaaaacaaacttcaggcatcatttaaatgccgagaattccaactcttcaagtcttgagagcttgccttaaaaatttccatagtggtatacaaaggactccagggtgctttcctgtggcttcaggaagggaagggaagacatttgccctgggtagtctgggacagtcccttgaaaagtctatttttgtttctctccccacttggattccaaaaagctagtgctggctccagtgccaccagaatactccaggccgttgggttttcaaatgtgagaggttgggtgatttcaagaatctatagagatttaaaatgtgcaatgaagccacaatttctgttcagatcctctgaaatatggggtgcaagaccccaattttgtgtggaatccttctcatgataaaaatattattctggatacttaggagatctgtgaccatcagcatctttataagaaagtgacctacaaaagctaccccaattttcaaatttgaaagttcagtggggagaaagtagtatggataatagtaatggttaccatagttaagattatccaattttcataatttctataaaaactttcaatgtgtaatccttatttgaaatagtatcaaaggaactataaaagaattttgttgttaacgtaactccgctctccagaaaatcaattagtgcaaatcatttgaagcaaaaaatcagaaccatttcactgagcaagtcttcagagattttttaaaaagaatatacaaatgcaaatttgttgtgcagtatataaaagggtggcaccccttttcacacttaaaatttcaggcatttacagctctgattccatttatagttaacaagaaaaatataaagtgttacttttttactgcaaaaataaggatcattagcaatctagaattcaaatacttaagaagccatatgtcaatattattaaactaattaattagctgtcaaaaccaatgaagattataatgatctagtgtctgacacatttgatctagggctgtgagaccactgggaattctacatattagacgagtaatttgtttgcactctgatactttcttctcataaaaatcacttgggaaccttgttaagaatgcaaattctgatttagtagacctagagtggcatgaaattctgcatttttaacaagataccagataatgccaatcctacttactggtcctcagaccacacagctagcaaaggtctagagaggtctaaatgaggttccattacagtgatagaacatgaaaatctgatctctcagctctgtcagctaacatttccccaaacttattctacaatgtttcctaagcacctcaacttgcttaaaatgccaatcttaaaatgccaaattagtttttaataataccaatactattaataactatgcacaggggaaattcattgttaaagaatgacaaaaagacatctgtaaattcacagtgatattttacaaatattttaaattgtacacagggttcctattaagttaatacaatatcaagtttcactgcccgattgccttacagttcttaactacaatttatggcaatagatcttattccattctgttactggagctaaaagaaaatcaaattcatttatgtcaaaatccacattgtaaacagggctaatgaatgaaaacgagttcatgctttttgaagaactcggtttaaactggtagccaaagcagttgcagttaaaactatgtccagagtataaatgctttggcagccttcaaagcatacaaatttttcatatatctgagctctgcataagcaggaacaagaggaaaacactagcatgctctcttggtgactacagcaagggactatgaagaaggaaaccgctgtgcagtcacagtgaaaaagagccaagaactggacagctccttaggtcttcctcaacggtcaactgactcagcctcagccgtgctttctctctctcactctgaatgatgacttaagtacatttgctttacaggggaaccgcaaccatagccaaaaggaccacggctagcaaacatcaaacttttatttccatctagaggtcacatacagatacatacaagtttgtttcaacttctgccatgtcgtctttttcatttttactttttagttgggaggtaactaaattgattattcttttgatatcatactaagatatttaaaacaggcctgttcactaacaagaaagacatttctttttcttcgtgttttaaatttaagaacacaaacataaacaactttagttaatatataaatgtcctttgtccatatttcactacctttattttctttcatgacattttatagatgaaaaatgcatttgcagacaaacaattacatattatacagtggtatcttgagagctatgttgcaagatttacactgatttccaggaagtcttccaatgacgtatgctctgaattataggagtccaaactaactaggatttccaaagtccagcagtagggtaaatcagctttacagcctattataccttaataattgaaagggatcttcacatgctaaatccagataaaacacttcaaaacaacacacctaccagcaatctgatttttgatataaaaatgtttcagagataacaacagaaatgcctctagccatcccctggaatcatataatattctaggcactgggttaccaggcattttccagggctttgagcaaattgttctaatcataaagatgatctgcttacaaatattttcatcaggtgcttttcatacacatcatttttgtgtttccacatgcctgttttcagattggcttcctgaccaggagctagagaattcctggagttgtgcctctgccccattctctataaaacagttcccatacatgcagactccctttgactctgaaggccaaacacacagccatcaaaataggagctattaaaaaaccaaaccaaaccaaaacaagaaaaaccaccttacaacctcacatgagacataaccaacttgattagacaacctgtcaaaatttattgtcactgacaatcttagggcaacaataacaaataagaggagggaaaaaaaagactcaaaccaaggggaaaaaatcttaatcaagaaataacaaaaccatatttcaacttactgcaacctagacaatcttcccttcataaagtcaggggagccttcagaatttaagacatcagggctcctgtcaggaatacggatgaaagacccagggtactttcataaagaagcaaagttgtatttccaggttcactaggttatgggagaaaaatatgttactaattaatctgtggacagagtaatgctaatactaggaggtctctgctgacctgattgatgcttcattggaagttcagttctttctgaaacgtaaataagcttttcttcttggagactacaagcggaaaacctattggcatctgtcccagccccacaaccaacagcagatgacgggttatgtgggactgtgacaccactgacttgttcaaaggatttactaaatacagtcgctgcggtcttagccaaaccatggctactaggcttaggtagggattggctggttgttaaagtaagtctcttcaaagagagaagctcaagattctcactttgggctctctgagtttgttttcgagcaaagtgatctttgcaagattcccctgtagtttctttttcttttcctccagttttgcttcctcctgaccgtctgtggttctttcctatacttggcttgttactacaattgtgactactgtttgataaacccgactggctggtactagacgcagccctggaataaaatccctcgtcaacttcagatatctccatcagttcttcttgacctgttaattctgtatttcagatttttgcctcctgatctctggcaagcctttgctctcagttctaggatctgtggctgtttcctgcacaccctgtatatgctgagcatcaatctctcctagtgttctgcctttttccccattcccggttctctctccggccacatttgtgacactaatctcaggaatgacaaggatgcccaattcagtagcatcattattgttgtcaggttgctcatgtcttttccacctatgaccccttattgacatgctggttactgcatttcttgatattcgagaggaagttggtgtgatttcaacttgaatacaccttgtaccttccttattagatttcatgggaccatgaggcaatgaagcctttattgcattagcaaccagcaatggctctggatataattctagctgggctctgtatataatatcatccagtgctttttgagctagatcccattctccattataaaaggcaaaataaatccctgttaacatttgcaccatgaatcctgaagaaactggtatcctgctacttatacctttatattttcttacatgttgtcgaggatatccacaaacacagattcttgaacaaatttgacacagtgactgaagagaaacactgggcatgtaagttaaggcagcattgtaacacaacaaaaggaatgtcaacacttcaaaccgattctgtgctgtcagcatctccctttgaggatgaggtccactgtataccacttttgacaaaccatgctgggatagtgcactctcagtcagagccatggacccaatgctggaaggttcatggtatacagatggtttggataaagatggaatcgtaaaactcaatactttggtatgtccctgtttgtcaactatttccaaattgtaaacccctagaagaagagcttcaatgcatccactgctatgcacatttctgctggctgagactgcaaggtagcaccaaattagttctgggagaaattgcagcgtaaattgaagcaactgctcctctccactgcgatagaattcaaagagctggtgacagacaggttctagcaactcactttgtggctcctggataactttatagagagatgaaactaaagaactcttgtctttcaaatttgtggcataatttggtaaagatgtttctggtaatgtcttaaactctgacaaccattcctccacaacccctttctctgaagtaaacatttttccacatctgttctaaaccttcaaccagggcggctgccggagctccacctgcaggacctcgactcgtgaggctctcagcgacagcgacggaggctgctctgcttcctcccgagtagcagcaccacctgctccccttcttcctagcagaacgggtcccggtgagccatcttccccctcctctcactgactgacaacccagccgggagagccaccactgccgccagcctctct

SEQ ID NO: 11385 - RNA, 7014 nt, Homo sapiens
  source 1..7014: mol_type = other RNA
ctgaatagctgggactacaggtgcccgccactatgcctggctaatttttgtatttttagtagagatggggtttcgccatgttggtcaggctggtcttgaactcctgacttcaggtgatccacccacctcggcctcccaaaaggctgggattacaggtgtgagccaccgcacccagccataagttcttttttctaagtacatgctataatgcaattcatgtaatgccactgagatttcctaaagccaacaaacaaaattctaaaattgtactgttaaagaaaacactgaagacttatccttgattcttttccaaagctaacatcaacctaactcatttattgtctcataaatgtctagatacctaccacgcacaaagtcctatctaggtactaggggcatataatctctgtactcaagagatatagactctttcttcttcttttgctttttttttttttttaagagataagatctcgttatattgcccaggctggtctcaaattcctgggctcgagtgaacctcctgagtagttgggactactactcaccacacatggcaataaagattctaaagttagaaggacaaagtgatgttacctaaatttgcctgtgcttctgatatgacaaataatccgccactggtgcatggcccatagagctcatcttcatctttggatgaatacgagtggacctgtcatactcctcagccctatgacatgtaaagcacaaagccaggaatgaggtcattgtcttatcacttacccccaaaagctctcaatggctcaacttacctaagtcttcctcctttattctcttccttcatatcaaaacttctgcaaatttttataataattttttaaatgagtaaactgatctggaaaaaatatttttttcagtttttatttcaataaaacaagaggcaacacttgttgtataaagtactacatatggagaacatttacacaaatatacaaaaattcaaaaaactaaactccagtttatttccatagccttaagaaggtagggaacacacaaaaatagccaaagtcgtcgtttattctttaggaatgtaaactctaggaatacaattagaaacaaatatatttactatgaaaagattagtatcactaaatgattagaaataaaggtaagaggtacacaataagttccatataagagaaagcaacaatacgtgaaataaaatcttgggtttatggtaaaaacttcctattaagacaaatgtactctaaaactctactataaaaaaacacaaaaacatctcccaaaatgttcgttgttagtttctttagatatgcacaagttacaaagtatagaagacaatatatttatgctctctgatgaagaatttaacaatattaaacataaatctgaataactcaaagtactgagtataattttactaagcaacaaatgtagaagtataaattcatgctcattaaaggactagagagttttaatttttcatacaaagactgggaggacactattatacattaatttctatctacaatgcttaaagtacccatcaaattatttttctttttaagtggtttttaaaaaatatttttcagttacattattcaacatgtatatatttccttgatgtgcttccctttaatacagatttattgtgcctaaacgcaaatgttaacctgccttattttaaatatttgtttaaaattatgtctcagagtacatctgttctctgtaattcaacagttttaacattttagttttattcttccaaaataggcaaaatcccttaaaactgggatcattttgatctattttggttttaaaaatatatttccctttaattcaactttttaaaaaaatgagtaatatttgctgagcagttgcttcacaattgaaaagagcaatgaaatattgctttttcaaaacaaacttcaggcatcatttaaatgccgagaattccaactcttcaagtcttgagagcttgccttaaaaatttccatagtggtatacaaaggactccagggtgctttcctgtggcttcaggaagggaagggaagacatttgccctgggtagtctgggacagtcccttgaaaagtctatttttgtttctctccccacttggattccaaaaagctagtgctggctccagtgccaccagaatactccaggccgttgggttttcaaatgtgagaggttgggtgatttcaagaatctatagagatttaaaatgtgcaatgaagccacaatttctgttcagatcctctgaaatatggggtgcaagaccccaattttgtgtggaatccttctcatgataaaaatattattctggatacttaggagatctgtgaccatcagcatctttataagaaagtgacctacaaaagctaccccaattttcaaatttgaaagttcagtggggagaaagtagtatggataatagtaatggttaccatagttaagattatccaattttcataatttctataaaaactttcaatgtgtaatccttatttgaaatagtatcaaaggaactataaaagaattttgttgttaacgtaactccgctctccagaaaatcaattagtgcaaatcatttgaagcaaaaaatcagaaccatttcactgagcaagtcttcagagattttttaaaaagaatatacaaatgcaaatttgttgtgcagtatataaaagggtggcaccccttttcacacttaaaatttcaggcatttacagctctgattccatttatagttaacaagaaaaatataaagtgttacttttttactgcaaaaataaggatcattagcaatctagaattcaaatacttaagaagccatatgtcaatattattaaactaattaattagctgtcaaaaccaatgaagattataatgatctagtgtctgacacatttgatctagggctgtgagaccactgggaattctacatattagacgagtaatttgtttgcactctgatactttcttctcataaaaatcacttgggaaccttgttaagaatgcaaattctgatttagtagacctagagtggcatgaaattctgcatttttaacaagataccagataatgccaatcctacttactggtcctcagaccacacagctagcaaaggtctagagaggtctaaatgaggttccattacagtgatagaacatgaaaatctgatctctcagctctgtcagctaacatttccccaaacttattctacaatgtttcctaagcacctcaacttgcttaaaatgccaatcttaaaatgccaaattagtttttaataataccaatactattaataactatgcacaggggaaattcattgttaaagaatgacaaaaagacatctgtaaattcacagtgatattttacaaatattttaaattgtacacagggttcctattaagttaatacaatatcaagtttcactgcccgattgccttacagttcttaactacaatttatggcaatagatcttattccattctgttactggagctaaaagaaaatcaaattcatttatgtcaaaatccacattgtaaacagggctaatgaatgaaaacgagttcatgctttttgaagaactcggtttaaactggtagccaaagcagttgcagttaaaactatgtccagagtataaatgctttggcagccttcaaagcatacaaatttttcatatatctgagctctgcataagcaggaacaagaggaaaacactagcatgctctcttggtgactacagcaagggactatgaagaaggaaaccgctgtgcagtcacagtgaaaaagagccaagaactggacagctccttaggtcttcctcaacggtcaactgactcagcctcagccgtgctttctctctctcactctgaatgatgacttaagtacatttgctttacaggggaaccgcaaccatagccaaaaggaccacggctagcaaacatcaaacttttatttccatctagaggtcacatacagatacatacaagtttgtttcaacttctgccatgtcgtctttttcatttttactttttagttgggaggtaactaaattgattattcttttgatatcatactaagatatttaaaacaggcctgttcactaacaagaaagacatttctttttcttcgtgttttaaatttaagaacacaaacataaacaactttagttaatatataaatgtcctttgtccatatttcactacctttattttctttcatgacattttatagatgaaaaatgcatttgcagacaaacaattacatattatacagtggtatcttgagagctatgttgcaagatttacactgatttccaggaagtcttccaatgacgtatgctctgaattataggagtccaaactaactaggatttccaaagtccagcagtagggtaaatcagctttacagcctattataccttaataattgaaagggatcttcacatgctaaatccagataaaacacttcaaaacaacacacctaccagcaatctgatttttgatataaaaatgtttcagagataacaacagaaatgcctctagccatcccctggaatcatataatattctaggcactgggttaccaggcattttccagggctttgagcaaattgttctaatcataaagatgatctgcttacaaatattttcatcaggtgcttttcatacacatcatttttgtgtttccacatgcctgttttcagattggcttcctgaccaggagctagagaattcctggagttgtgcctctgccccattctctataaaacagttcccatacatgcagactccctttgactctgaaggccaaacacacagccatcaaaataggagctattaaaaaaccaaaccaaaccaaaacaagaaaaaccaccttacaacctcacatgagacataaccaacttgattagacaacctgtcaaaatttattgtcactgacaatcttagggcaacaataacaaataagaggagggaaaaaaaagactcaaaccaaggggaaaaaatcttaatcaagaaataacaaaaccatatttcaacttactgcaacctagacaatcttcccttcataaagtcaggggagccttcagaatttaagacatcagggctcctgtcaggaatacggatgaaagacccagggtactttcataaagaagcaaagttgtatttccaggttcactaggttatgggagaaaaatatgttactaattaatctgtggacagagtaatgctaatactaggaggtctctgctgacctgattgatgcttcattggaagttcagttctttctgaaacgtaaataagcttttcttcttggagactacaagcggaaaacctattggcatctgtcccagccccacaaccaacagcagatgacgggttatgtgggactgtgacaccactgacttgttcaaaggatttactaaatacagtcgctgcggtcttagccaaaccatggctactaggcttaggtagggattggctggttgttaaagtaagtctcttcaaagagagaagctcaagattctcactttgggctctctgagtttgttttcgagcaaagtgatctttgcaagattcccctgtagtttctttttcttttcctccagttttgcttcctcctgaccgtctgtggttctttcctatacttggcttgttactacaattgtgactactgtttgataaacccgactggctggtactagacgcagccctggaataaaatccctcgtcaacttcagatatctccatcagttcttcttgacctgttaattctgtatttccatgtcttttccacctatgaccccttattgacatgctggttactgcatttcttgatattcgagaggaagttggtgtgatttcaacttgaatacaccttgtaccttccttattagatttcatgggaccatgaggcaatgaagcctttattgcattagcaaccagcaatggctctggatataattctagctgggctctgtatataatatcatccagtgctttttgagctagatcccattctccattataaaaggcaaaataaatccctgttaacatttgcaccatgaatcctgaagaaactggtatcctgctacttatacctttatattttcttacatgttgtcgaggatatccacaaacacagattcttgaacaaatttgacacagtgactgaagagaaacactgggcatgtaagttaaggcagcattgtaacacaacaaaaggaatgtcaacacttcaaaccgattctgtgctgtcagcatctccctttgaggatgaggtccactgtataccacttttgacaaaccatgctgggatagtgcactctcagtcagagccatggacccaatgctggaaggttcatggtatacagatggtttggataaagatggaatcgtaaaactcaatactttggtatgtccctgtttgtcaactatttccaaattgtaaacccctagaagaagagcttcaatgcatccactgctatgcacatttctgctggctgagactgcaaggtagcaccaaattagttctgggagaaattgcagcgtaaattgaagcaactgctcctctccactgcgatagaattcaaagagctggtgacagacaggttctagcaactcactttgtggctcctggataactttatagagagatgaaactaaagaactcttgtctttcaaatttgtggcataatttggtaaagatgtttctggtaatgtcttaaactctgacaaccattcctccacaacccctttctctgaagtaaacatttttccacatctgttctaaaccttcaaccagggcggctgccggagctccacctgcaggacctcgactcgtgaggctctcagcgacagcgacggaggctgctctgcttcctcccgagtagcagcaccacctgctccccttcttcctagcagaacgggtcccggtgagccatcttccccctcctctcactgactgacaacccagccgggagagccaccactgccgccagcctctct

SEQ ID NO: 11386 - RNA, 7310 nt, Homo sapiens
  source 1..7310: mol_type = other RNA
ctgaatagctgggactacaggtgcccgccactatgcctggctaatttttgtatttttagtagagatggggtttcgccatgttggtcaggctggtcttgaactcctgacttcaggtgatccacccacctcggcctcccaaaaggctgggattacaggtgtgagccaccgcacccagccataagttcttttttctaagtacatgctataatgcaattcatgtaatgccactgagatttcctaaagccaacaaacaaaattctaaaattgtactgttaaagaaaacactgaagacttatccttgattcttttccaaagctaacatcaacctaactcatttattgtctcataaatgtctagatacctaccacgcacaaagtcctatctaggtactaggggcatataatctctgtactcaagagatatagactctttcttcttcttttgctttttttttttttttaagagataagatctcgttatattgcccaggctggtctcaaattcctgggctcgagtgaacctcctgagtagttgggactactactcaccacacatggcaataaagattctaaagttagaaggacaaagtgatgttacctaaatttgcctgtgcttctgatatgacaaataatccgccactggtgcatggcccatagagctcatcttcatctttggatgaatacgagtggacctgtcatactcctcagccctatgacatgtaaagcacaaagccaggaatgaggtcattgtcttatcacttacccccaaaagctctcaatggctcaacttacctaagtcttcctcctttattctcttccttcatatcaaaacttctgcaaatttttataataattttttaaatgagtaaactgatctggaaaaaatatttttttcagtttttatttcaataaaacaagaggcaacacttgttgtataaagtactacatatggagaacatttacacaaatatacaaaaattcaaaaaactaaactccagtttatttccatagccttaagaaggtagggaacacacaaaaatagccaaagtcgtcgtttattctttaggaatgtaaactctaggaatacaattagaaacaaatatatttactatgaaaagattagtatcactaaatgattagaaataaaggtaagaggtacacaataagttccatataagagaaagcaacaatacgtgaaataaaatcttgggtttatggtaaaaacttcctattaagacaaatgtactctaaaactctactataaaaaaacacaaaaacatctcccaaaatgttcgttgttagtttctttagatatgcacaagttacaaagtatagaagacaatatatttatgctctctgatgaagaatttaacaatattaaacataaatctgaataactcaaagtactgagtataattttactaagcaacaaatgtagaagtataaattcatgctcattaaaggactagagagttttaatttttcatacaaagactgggaggacactattatacattaatttctatctacaatgcttaaagtacccatcaaattatttttctttttaagtggtttttaaaaaatatttttcagttacattattcaacatgtatatatttccttgatgtgcttccctttaatacagatttattgtgcctaaacgcaaatgttaacctgccttattttaaatatttgtttaaaattatgtctcagagtacatctgttctctgtaattcaacagttttaacattttagttttattcttccaaaataggcaaaatcccttaaaactgggatcattttgatctattttggttttaaaaatatatttccctttaattcaactttttaaaaaaatgagtaatatttgctgagcagttgcttcacaattgaaaagagcaatgaaatattgctttttcaaaacaaacttcaggcatcatttaaatgccgagaattccaactcttcaagtcttgagagcttgccttaaaaatttccatagtggtatacaaaggactccagggtgctttcctgtggcttcaggaagggaagggaagacatttgccctgggtagtctgggacagtcccttgaaaagtctatttttgtttctctccccacttggattccaaaaagctagtgctggctccagtgccaccagaatactccaggccgttgggttttcaaatgtgagaggttgggtgatttcaagaatctatagagatttaaaatgtgcaatgaagccacaatttctgttcagatcctctgaaatatggggtgcaagaccccaattttgtgtggaatccttctcatgataaaaatattattctggatacttaggagatctgtgaccatcagcatctttataagaaagtgacctacaaaagctaccccaattttcaaatttgaaagttcagtggggagaaagtagtatggataatagtaatggttaccatagttaagattatccaattttcataatttctataaaaactttcaatgtgtaatccttatttgaaatagtatcaaaggaactataaaagaattttgttgttaacgtaactccgctctccagaaaatcaattagtgcaaatcatttgaagcaaaaaatcagaaccatttcactgagcaagtcttcagagattttttaaaaagaatatacaaatgcaaatttgttgtgcagtatataaaagggtggcaccccttttcacacttaaaatttcaggcatttacagctctgattccatttatagttaacaagaaaaatataaagtgttacttttttactgcaaaaataaggatcattagcaatctagaattcaaatacttaagaagccatatgtcaatattattaaactaattaattagctgtcaaaaccaatgaagattataatgatctagtgtctgacacatttgatctagggctgtgagaccactgggaattctacatattagacgagtaatttgtttgcactctgatactttcttctcataaaaatcacttgggaaccttgttaagaatgcaaattctgatttagtagacctagagtggcatgaaattctgcatttttaacaagataccagataatgccaatcctacttactggtcctcagaccacacagctagcaaaggtctagagaggtctaaatgaggttccattacagtgatagaacatgaaaatctgatctctcagctctgtcagctaacatttccccaaacttattctacaatgtttcctaagcacctcaacttgcttaaaatgccaatcttaaaatgccaaattagtttttaataataccaatactattaataactatgcacaggggaaattcattgttaaagaatgacaaaaagacatctgtaaattcacagtgatattttacaaatattttaaattgtacacagggttcctattaagttaatacaatatcaagtttcactgcccgattgccttacagttcttaactacaatttatggcaatagatcttattccattctgttactggagctaaaagaaaatcaaattcatttatgtcaaaatccacattgtaaacagggctaatgaatgaaaacgagttcatgctttttgaagaactcggtttaaactggtagccaaagcagttgcagttaaaactatgtccagagtataaatgctttggcagccttcaaagcatacaaatttttcatatatctgagctctgcataagcaggaacaagaggaaaacactagcatgctctcttggtgactacagcaagggactatgaagaaggaaaccgctgtgcagtcacagtgaaaaagagccaagaactggacagctccttaggtcttcctcaacggtcaactgactcagcctcagccgtgctttctctctctcactctgaatgatgacttaagtacatttgctttacaggggaaccgcaaccatagccaaaaggaccacggctagcaaacatcaaacttttatttccatctagaggtcacatacagatacatacaagtttgtttcaacttctgccatgtcgtctttttcatttttactttttagttgggaggtaactaaattgattattcttttgatatcatactaagatatttaaaacaggcctgttcactaacaagaaagacatttctttttcttcgtgttttaaatttaagaacacaaacataaacaactttagttaatatataaatgtcctttgtccatatttcactacctttattttctttcatgacattttatagatgaaaaatgcatttgcagacaaacaattacatattatacagtggtatcttgagagctatgttgcaagatttacactgatttccaggaagtcttccaatgacgtatgctctgaattataggagtccaaactaactaggatttccaaagtccagcagtagggtaaatcagctttacagcctattataccttaataattgaaagggatcttcacatgctaaatccagataaaacacttcaaaacaacacacctaccagcaatctgatttttgatataaaaatgtttcagagataacaacagaaatgcctctagccatcccctggaatcatataatattctaggcactgggttaccaggcattttccagggctttgagcaaattgttctaatcataaagatgatctgcttacaaatattttcatcaggtgcttttcatacacatcatttttgtgtttccacatgcctgttttcagattggcttcctgaccaggagctagagaattcctggagttgtgcctctgccccattctctataaaacagttcccatacatgcagactccctttgactctgaaggccaaacacacagccatcaaaataggagctattaaaaaaccaaaccaaaccaaaacaagaaaaaccaccttacaacctcacatgagacataaccaacttgattagacaacctgtcaaaatttattgtcactgacaatcttagggcaacaataacaaataagaggagggaaaaaaaagactcaaaccaaggggaaaaaatcttaatcaagaaataacaaaaccatatttcaacttactgcaacctagacaatcttcccttcataaagtcaggggagccttcagaatttaagacatcagggctcctgtcaggaatacggatgaaagacccagggtactttcataaagaagcaaagttgtatttccaggttcactaggttatgggagaaaaatatgttactaattaatctgtggacagagtaatgctaatactaggaggtctctgctgacctgattgatgcttcattggaagttcagttctttctgaaacgtaaataagcttttcttcttggagactacaagcggaaaacctattggcatctgtcccagccccacaaccaacagcagatgacgggttatgtgggactgtgacaccactgacttgttcaaaggatttactaaatacagtcgctgcggtcttagccaaaccatggctactaggcttaggtagggattggctggttgttaaagtaagtctcttcaaagagagaagctcaagattctcactttgggctctctgagtttgttttcgagcaaagtgatctttgcaagattcccctgtagtttctttttcttttcctccagttttgcttcctcctgaccgtctgtggttctttcctatacttggcttgttactacaattgtgactactgtttgataaacccgactggctggtactagacgcagccctggaataaaatccctcgtcaacttcagatatctccatcagttcttcttgacctgttaattctgtatttccttggagtgcagttataaagtgctctgctaaaactgcactctgccaggtgagtttattccatcctccatcatttttcttacagatttttgcctcctgatctctggcaagcctttgctctcagttctaggatctgtggctgtttcctgcacaccctgtatatgctgagcatcaatctctcctagtgttctgcctttttccccattcccggttctctctccggccacatttgtgacactaatctcaggaatgacaaggatgcccaattcagtagcatcattattgttgtcaggttgctcatgtcttttccacctatgaccccttattgacatgctggttactgcatttcttgatattcgagaggaagttggtgtgatttcaacttgaatacaccttgtaccttccttattagatttcatgggaccatgaggcaatgaagcctttattgcattagcaaccagcaatggctctggatataattctagctgggctctgtatataatatcatccagtgctttttgagctagatcccattctccattataaaaggcaaaataaatccctgttaacatttgcaccatgaatcctgaagaaactggtatcctgctacttatacctttatattttcttacatgttgtcgaggatatccacaaacacagattcttgaacaaatttgacacagtgactgaagagaaacactgggcatgtaagttaaggcagcattgtaacacaacaaaaggaatgtcaacacttcaaaccgattctgtgctgtcagcatctccctttgaggatgaggtccactgtataccacttttgacaaaccatgctgggatagtgcactctcagtcagagccatggacccaatgctggaaggttcatggtatacagatggtttggataaagatggaatcgtaaaactcaatactttggtatgtccctgtttgtcaactatttccaaattgtaaacccctagaagaagagcttcaatgcatccactgctatgcacatttctgctggctgagactgcaaggtagcaccaaattagttctgggagaaattgcagcgtaaattgaagcaactgctcctctccactgcgatagaattcaaagagctggtgacagacaggttctagcaactcactttgtggctcctggataactttatagagagatgaaactaaagaactcttgtctttcaaatttgtggcataatttggtaaagatgtttctggtaatgtcttaaactctgacaaccattcctccacaacccctttctctgaagtaaacatttttccacatctgttctaaaccttcaaccagggcggctgccggagctccacctgcaggacctcgactcgtgaggctctcagcgacagcgacggaggctgctctgcttcctcccgagtagcagcaccacctgctccccttcttcctagcagaacgggtcccggtgagccatcttccccctcctctcactgactgacaacccagccgggagagccaccactgccgccagcctctct

SEQ ID NO: 11387 - RNA, 2460 nt, Homo sapiens
  source 1..2460: mol_type = other RNA
ctgaatagctgggactacaggtgcccgccatcacgcccggctaattttttttttttttttgagatggagtctggctctgtcgcccaggctggagtgcagtggcgccatctcagctcactgcaagctctgcctcccgggttcacgccattgccattctcccgcctcagcctcccaagtagctggggctacaggcgcccgccaccacgcccagctaattttctgtatttttttagtagagacagggtttcaccatgttggccaggctggtctcgaactcctgacctcaagtgatccgcccacctaggcctcccaaagtgctgggattacaggcgtgagtcactgcgcccggccccagtgactatttatgagaacaaaagacaaggcatggctgactctccaggttacagctggagaagaggggaaaggtgtttggttgtacaagcagctcagggcagctggtgctgcggcgtgcatgtgcggcccgagagcgtggcttcgggtctaccagatgccttcaaggaaaaggccagaacctgcactgcacggcacagtcactgtgtgtggtgggacccagtgtcggctgagaggcctggaggggtcttgcctcccttgtagtcacttggtgtcataacaaggagggcactcatttggcctgggccggcccctggccccactatccacaggccaggcccggccaatgaccttgcctaggcaggaagtcccccaggctgtcccctcgctgcctagggccatgggcaagctgcacaggctccggggcctgagccagagcccccgcctcctgctgccacagcccaagggagtggctgagtcagccttagaggccattctgtggccgagagctggaggccagtggctgcggggggtgggggaggggtcctttccccaccccggtggcccctctgagtccgtgtggccagggctctggctgggaaaagagaatttgagcctagcgtactttgcagcagccctcaaataactcagcctcctcaagggggcatctgatagatgcccgtgaacatgtcttctccggcctggccaggctgcccaccattggaaacatcccccagggcctgaccccactgccgagggctgcagcaccccccacacctgctgggctgacgtgtgtcctggctcctgtcttcccctgaagccaggccacccagctccctccagggccaggcagggaagcaccaagccctggcgtgcacctgcacccactcaaacgccgaagccttcgtgtcatcactgtcacacgggccactcagcacccatgaagtccaccacgggtctctggggcaatccttctctgaacgcaaaaccctgccctggctctcccaggtctgccagccacgcatgccgggtctgagactcccccggaccgctgggtgctgcttggagcccctcctggcccaggactgatgggcaggtcccgctggagcctcttcaccgtgtccccgacccaggaaaccccgaggccaaggaaccagcctggctttgcccccaacgctcttagcaacacagtccctcattgaaccaaacggttctatctcaggagaagtcatccagtccttatggtattaagacaagaggaaaactttggtcttgaactacccggcagccttgcaaaatgtctgcatctgacaaatccccgcctctgcggactcccgggcacagggccgctcccagccccggccctcggcccctcacaagacctgcaggctgcgctcatgcccgtccagctggaccttgagcttgtggagctcctcgatctcgcggttgtggcgctccgttttgtggcgcaccagggagcggtagaagtggatggtgaagaccacgaagatgaggcccacgggcaccatgatgatggtggacaccagggcggcctgccagcccgtgtgactcccagggccaggtggggggccaggctggcgccgggcatccacggggaggaacttgatccagcagagcagcaccacctcggccaggaagagtaggatgccaagcacggtggagaagccccaggccagctcgatgtaggggtgcatgcgctcatgcggggactcgctgatggagttcaggttgtggatgttgctcacggcctccacattgggcaggatgcaggtgctgatgaggagggcgaacaggtgcacggccaccagcaccgtggtgcaggcgctgaaggcaatcagcagcggccgcgggtactggtactgcgtctccagctgcacctccaccatggccaccaggtcatttatacgaatgccaactcaggctctccatcccatctccttgcgcacatccgcagccagcagcaccgcatccaagcacttccatccctgggacgttccttcccggagctgccctcgccccgcccggctcggctcccgctcggactgcgtggccgcgtggcctgtggcccagtggcccggccggggcgcc

SEQ ID NO: 11388 - RNA, 2698 nt, Homo sapiens
  source 1..2698: mol_type = other RNA
ctgaatagctgggactacaggtgcccgccatcacgcccggctaattttttttttttttttgagatggagtctggctctgtcgcccaggctggagtgcagtggcgccatctcagctcactgcaagctctgcctcccgggttcacgccattgccattctcccgcctcagcctcccaagtagctggggctacaggcgcccgccaccacgcccagctaattttctgtatttttttagtagagacagggtttcaccatgttggccaggctggtctcgaactcctgacctcaagtgatccgcccacctaggcctcccaaagtgctgggattacaggcgtgagtcactgcgcccggccccagtgactatttatgagaacaaaagacaaggcatggctgactctccaggttacagctggagaagaggggaaaggtgtttggttgtacaagcagctcagggcagctggtgctgcggcgtgcatgtgcggcccgagagcgtggcttcgggtctaccagatgccttcaaggaaaaggccagaacctgcactgcacggcacagtcactgtgtgtggtgggacccagtgtcggctgagaggcctggaggggtcttgcctcccttgtagtcacttggtgtcataacaaggagggcactcatttggcctgggccggcccctggccccactatccacaggccaggcccggccaatgaccttgcctaggcaggaagtcccccaggctgtcccctcgctgcctagggccatgggcaagctgcacaggctccggggcctgagccagagcccccgcctcctgctgccacagcccaagggagtggctgagtcagccttagaggccattctgtggccgagagctggaggccagtggctgcggggggtgggggaggggtcctttccccaccccggtggcccctctgagtccgtgtggccagggctctggctgggaaaagagaatttgagcctagcgtactttgcagcagccctcaaataactcagcctcctcaagggggcatctgatagatgcccgtgaacatgtcttctccggcctggccaggctgcccaccattggaaacatcccccagggcctgaccccactgccgagggctgcagcaccccccacacctgctgggctgacgtgtgtcctggctcctgtcttcccctgaagccaggccacccagctccctccagggccaggcagggaagcaccaagccctggcgtgcacctgcacccactcaaacgccgaagccttcgtgtcatcactgtcacacgggccactcagcacccatgaagtccaccacgggtctctggggcaatccttctctgaacgcaaaaccctgccctggctctcccaggtctgccagccacgcatgccgggtctgagactcccccggaccgctgggtgctgcttggagcccctcctggcccaggactgatgggcaggtcccgctggagcctcttcaccgtgtccccgacccaggaaaccccgaggccaaggaaccagcctggctttgcccccaacgctcttagcaacacagtccctcattgaaccaaacggttctatctcaggagaagtcatccagtccttatggtattaagacaagaggaaaactttggtcttgaactacccggcagccttgcaaaatgtctgcatctgacaaatccccgcctctgcggactcccgggcacagggccgctcccagccccggccctcggcccctcacaagacctgcaggctgcgctcatgcccgtccagctggaccttgagcttgtggagctcctcgatctcgcggttgtggcgctccgttttgtggcgcaccagggagcggtagaagtggatggtgaagaccacgaagatgaggcccacgggcaccatgatgatggtggacaccagggcggcctgccagcccgtgtgactcccagggccaggtggggggccaggctggcgccgggcatccacggggaggaacttgatccagcagagcagcaccacctcggccaggaagagtaggatgccaagcacggtggagaagccccaggccagctcgatgtaggggtgcatgcgctcatgcggggactcgctgatggagttcaggttgtggatgttgctcacggcctccacattgggcaggatgcaggtgctgatgaggagggcgaacaggtgcacggccaccagcaccgtggtgcaggcgctgaaggcaatcagcagcggccgcgggtactggtactgcgtctccagctgcacctccaccatggccaccatggcaaagccggagaggagggcggaggtcctgctggaggccttcagcttggccctgctcaggtagagcttccgccacgacagggcctgtaccgagtggtggttagaggtgaccagttccaggtagctgcggcggacccagtcccggtaatccatgcccttatggccgggctcagggcaggcaggagcagaggggtcgataggcacgttaagctcagcactcatggtgggagccaggcaggtcatttatacgaatgccaactcaggctctccatcccatctccttgcgcacatccgcagccagcagcaccgcatccaagcacttccatccctgggacgttccttcccggagctgccctcgccccgcccggctcggctcccgctcggactgcgtggccgcgtggcctgtggcccagtggcccggccggggcgcc

SEQ ID NO: 11389 - RNA, 2721 nt, Homo sapiens
  source 1..2721: mol_type = other RNA
ctgaatagctgggactacaggtgcccgccatcacgcccggctaattttttttttttttttgagatggagtctggctctgtcgcccaggctggagtgcagtggcgccatctcagctcactgcaagctctgcctcccgggttcacgccattgccattctcccgcctcagcctcccaagtagctggggctacaggcgcccgccaccacgcccagctaattttctgtatttttttagtagagacagggtttcaccatgttggccaggctggtctcgaactcctgacctcaagtgatccgcccacctaggcctcccaaagtgctgggattacaggcgtgagtcactgcgcccggccccagtgactatttatgagaacaaaagacaaggcatggctgactctccaggttacagctggagaagaggggaaaggtgtttggttgtacaagcagctcagggcagctggtgctgcggcgtgcatgtgcggcccgagagcgtggcttcgggtctaccagatgccttcaaggaaaaggccagaacctgcactgcacggcacagtcactgtgtgtggtgggacccagtgtcggctgagaggcctggaggggtcttgcctcccttgtagtcacttggtgtcataacaaggagggcactcatttggcctgggccggcccctggccccactatccacaggccaggcccggccaatgaccttgcctaggcaggaagtcccccaggctgtcccctcgctgcctagggccatgggcaagctgcacaggctccggggcctgagccagagcccccgcctcctgctgccacagcccaagggagtggctgagtcagccttagaggccattctgtggccgagagctggaggccagtggctgcggggggtgggggaggggtcctttccccaccccggtggcccctctgagtccgtgtggccagggctctggctgggaaaagagaatttgagcctagcgtactttgcagcagccctcaaataactcagcctcctcaagggggcatctgatagatgcccgtgaacatgtcttctccggcctggccaggctgcccaccattggaaacatcccccagggcctgaccccactgccgagggctgcagcaccccccacacctgctgggctgacgtgtgtcctggctcctgtcttcccctgaagccaggccacccagctccctccagggccaggcagggaagcaccaagccctggcgtgcacctgcacccactcaaacgccgaagccttcgtgtcatcactgtcacacgggccactcagcacccatgaagtccaccacgggtctctggggcaatccttctctgaacgcaaaaccctgccctggctctcccaggtctgccagccacgcatgccgggtctgagactcccccggaccgctgggtgctgcttggagcccctcctggcccaggactgatgggcaggtcccgctggagcctcttcaccgtgtccccgacccaggaaaccccgaggccaaggaaccagcctggctttgcccccaacgctcttagcaacacagtccctcattgaaccaaacggttctatctcaggagaagtcatccagtccttatggtattaagacaagaggaaaactttggtcttgaactacccggcagccttgcaaaatgtctgcatctgacaaatccccgcctctgcggactcccgggcacagggccgctcccagccccggccctcggcccctcacaagacctgcaggctgcgctcatgcccgtccagctggaccttgagcttgtggagctcctcgatctcgcggttgtggcgctccgttttgtggcgcaccagggagcggtagaagtggatggtgaagaccacgaagatgaggcccacgggcaccatgatgatggtggacaccagggcggcctgccagcccgtgtgactcccagggccaggtggggggccaggctggcgccgggcatccacggggaggaacttgatccagcagagcagcaccacctcggccaggaagagtaggatgccaagcacggtggagaagccccaggccagctcgatgtaggggtgcatgcgctcatgcggggactcgctgatggagttcaggttgtggatgttgctcacggcctccacattgggcaggatgcaggtgctgatgaggagggcgaacaggtgcacggccaccagcaccgtggtgcaggcgctgaaggcaatcagcagcggccgcgggtactggtactgcgtctccagctgcacctccaccatggccaccatggcaaagccggagaggagggcggaggtcctgctggaggccttcagcttggccctgctcaggtagagcttccgccacgacagggcctgtaccgagtggtggttagaggtgaccagttccaggtagctgcggcggacccagtcccggtaatccatgcccttatggccgggctcagggcaggcaggagcagaggggtcgataggcacgttaagctcagcactcatggtgggagccaggcaggtcatttatacgaatgccaactcaggctctccatcccatctccttgcgcacatccgcagccagcagcaccgcatccaagcacttccatccctgggacgttccttcccttggggagaattcagagaaacgcggagctgccctcgccccgcccggctcggctcccgctcggactgcgtggccgcgtggcctgtggcccagtggcccggccggggcgcc

SEQ ID NO: 11390 - RNA, 2589 nt, Homo sapiens
  source 1..2589: mol_type = other RNA
ctgaatagctgggactacaggtgcccgccatcacgcccggctaattttttttttttttttgagatggagtctggctctgtcgcccaggctggagtgcagtggcgccatctcagctcactgcaagctctgcctcccgggttcacgccattgccattctcccgcctcagcctcccaagtagctggggctacaggcgcccgccaccacgcccagctaattttctgtatttttttagtagagacagggtttcaccatgttggccaggctggtctcgaactcctgacctcaagtgatccgcccacctaggcctcccaaagtgctgggattacaggcgtgagtcactgcgcccggccccagtgactatttatgagaacaaaagacaaggcatggctgactctccaggttacagctggagaagaggggaaaggtgtttggttgtacaagcagctcagggcagctggtgctgcggcgtgcatgtgcggcccgagagcgtggcttcgggtctaccagatgccttcaaggaaaaggccagaacctgcactgcacggcacagtcactgtgtgtggtgggacccagtgtcggctgagaggcctggaggggtcttgcctcccttgtagtcacttggtgtcataacaaggagggcactcatttggcctgggccggcccctggccccactatccacaggccaggcccggccaatgaccttgcctaggcaggaagtcccccaggctgtcccctcgctgcctagggccatgggcaagctgcacaggctccggggcctgagccagagcccccgcctcctgctgccacagcccaagggagtggctgagtcagccttagaggccattctgtggccgagagctggaggccagtggctgcggggggtgggggaggggtcctttccccaccccggtggcccctctgagtccgtgtggccagggctctggctgggaaaagagaatttgagcctagcgtactttgcagcagccctcaaataactcagcctcctcaagggggcatctgatagatgcccgtgaacatgtcttctccggcctggccaggctgcccaccattggaaacatcccccagggcctgaccccactgccgagggctgcagcaccccccacacctgctgggctgacgtgtgtcctggctcctgtcttcccctgaagccaggccacccagctccctccagggccaggcagggaagcaccaagccctggcgtgcacctgcacccactcaaacgccgaagccttcgtgtcatcactgtcacacgggccactcagcacccatgaagtccaccacgggtctctggggcaatccttctctgaacgcaaaaccctgccctggctctcccaggtctgccagccacgcatgccgggtctgagactcccccggaccgctgggtgctgcttggagcccctcctggcccaggactgatgggcaggtcccgctggagcctcttcaccgtgtccccgacccaggaaaccccgaggccaaggaaccagcctggctttgcccccaacgctcttagcaacacagtccctcattgaaccaaacggttctatctcaggagaagtcatccagtccttatggtattaagacaagaggaaaactttggtcttgaactacccggcagccttgcaaaatgtctgcatctgacaaatccccgcctctgcggactcccgggcacagggccgctcccagccccggccctcggcccctcacaagacctgcaggctgcgctcatgcccgtccagctggaccttgagcttgtggagctcctcgatctcgcggttgtggcgctccgttttgtggcgcaccagggagcggtagaagtggatggtgaagaccacgaagatgaggcccacgggcaccatgatgatggtggacaccagggcggcctgccagcccgtgtgactcccagggccaggtggggggccaggctggcgccgggcatccacggggaggaacttgatccagcagagcagcaccacctcggccaggaagagtaggatgccaagcacggtggagaagccccaggccagctcgatgtaggggtgcatgcgctcatgcggggactcgctgatggagttcaggttgtggatgttgctcacggcctccacattgggcaggatgcaggtgctgatgaggagggcgaacaggtgcacggccaccagcaccgtggtgcaggcgctgaaggcaatcagcagcggccgcgggtactggtactgcgtctccagctgcacctccaccatggccaccatggcaaagccggagaggagggcggaggtcctgctggaggccttcagcttggccctgctcaggtagagcttccgccacgacagggcctgtaccgagtggtggttagaggtgaccagttccaggtagctgcggcggacccagtcccggtaatccatgcccttatggccgggctcagggcaggcaggagcagaggggtcgataggcacgttaagctcagcactcatggtgggagccaggcggagctgccctcgccccgcccggctcggctcccgctcggactgcgtggccgcgtggcctgtggcccagtggcccggccggggcgcc

SEQ ID NO: 11391 - RNA, 2592 nt, Homo sapiens
  source 1..2592: mol_type = other RNA
ctgaatagctgggactacaggtgcccgccatcatgcccggctaattctttttgtacttttagtagagatggggtttcaccgtgttagccaggatggtcttgatctcctgaacatagtcccatttcttaaaagctcacatcgtagccagggatatgtattgactttatatagatacatattgattatagcttgtgctgaacgttaaagcagaaagatgtggaagtgtgtcagtgaccaggtcacgaaatccaagcaagaatgatgatgatgagattcggagttttagaggtaatccaagaagtaaaacacaaaaaaagcaagaaaatggaggacctgcgcaacttcctgtagatagtatacaggtattccttgtgaaacatcagacctcagagttacttctggagtttttcttgtggcagagtttgaagattgcagcctgtgaaaactttaaaaacagtggaaagtccagatcctggtgtgttgtactcttgggtctgatggtcttctgcaatctgaggtctacctctgtagtcccagatactcgagaagctgaggagggaggatggctttaatccaggagttagacaccagcctgtgctggacagcataacaataccttattttggttttgtatttttctgttcctacaattgaatttttgagacactggaaggtaactctttaatcacctgagttgcaaatgtggtactaacaattcagtgtcacaagtgcttttcaaagtatgttaagctttttgttgatgtcatgtcaggcatatggtaattgtctgggtcaccactataatattccttatttggaatgtggtttcctagcaactcttgctttttcctaatggctgaattgatttctggacatttgtaatgcttcctactgcatcagaaattgtcaccttgtgtgtaaatgttacaagaccaaatttacatgtagattccattttaagaaattattttgctttatcacttgcctttaatgtgtttgttcagaggttaaaccaatcaatcataaaaaatgaatttagaaaacctcattaattcagactctttagggaaatatggtaattttgacaaattccaaaatatatgcaaatagttcttagtggggaacctcctgaagttgaagaaacagagtaattttgatggtcaaatgaccatgtaatcaggaggttgttagaaacacaggtccggagtatgcatggggtgtcccaggggagaaaaggcttactttggaggcttgctgtttcaactcacatgaagcctgattctacatgaatctggttggagccttgctggcagcgacttttactcatttattcaacaaatgttttttgaatgcttatgattttctaaacaattggttaggtattagaaatgtgagggtaagcaaaccaggtacatccctgatcctcccacgaattacagcctatggaaccaacaactagaaattactaacttggtgaggaaggagaaatagactcagttttctctcaatactctttccaccttaacatcgagaggtttgggttaggcttttaggaatataattctttgtagagcaaatattcaggatgtcatttacattcagacctacattattttggtgtttttgtagatttcatatgttcttagggaagtgaggttgaaaggcattaaaaaccaactatgtggtaggggttagcttgacatttacatattatctcacttaatctacacaacaactaagaagggcatatatgcaatttttatatacttaaaagataaaaaaagacattggggttaaaaatatgtacaagattatagaggaaaaaatgcatactggacactttccagatgtcagacttgtgccatgtctttatgcactatttattcctgccccccaacccccccccaaaaaaatctgcaaagtaagtttcgttaatcttattttacatttaaagaatttgagatttagaaagtttatataatttgatcaaggttatgtagctagccaattgcagaactaaatttgaatccagatatatctgtttggaaaaaagaaaaaagctttgctttttttcagtataggaaactggagaatgcccagagtagaattttattacctgagtacttaataacaagagttacttctcacctagtgcttactacgtgctcagcattatgccaagctagagtgcgtgagcactctctctcttacatgtcctctcccttcctaatatatatgcatatacacatacacctgtataattatttacatgtatgtgtatattttaggcatattttcatatttgtgaaatatgcctgtactgtatatacataattattacaacaatcatggaccatggattagatgttatctctatttataaatgggaaaaccaagactgaaaggttaagggactttttgtcaagagtaaataatattactaagtaagaattgattcggaattggaattcaaatctgtttgacttcaaagtccatgctcgtaaccattaccctatactgccactcacaatacaactggaatgtattaatatgatttctaatcttatgactaagctaataactttaattttc

SEQ ID NO: 11392 - RNA, 8386 nt, Homo sapiens
  source 1..8386: mol_type = other RNA
ctgaatagctgggactacaggtgcccgccgccacacctggctaactttttgtattttttagtagagacagggtttcactatgttagccaggatggtcttgatctcctgacctcgtgatctgcccacctcggcctcccaaagtgctgggattacaagcgtgagccaccatgcccggcctcctctgggtagttctgagaaaagggctgtctctgtgacagaaacatagctctttctaaatgccctgatgcatgactgacttattctccctccctcattctttcccgatgaactgaaaggtcttccatgctctgttcaaattgaatgttggccaacatcactctcattcctcctcctggcaagaatggcatcctagggtcctagggcccgcgagtgatgcaagaattctaaaacctagtttcaaaagagtacctactaaagatttcattcactttcttgtggttctagtaaggattaatgttgaataagaagagacacacattagaatgtacatatacatacacatagaatatcctcctgttctaaatccacatgagaacacaggcaggcctacacttgagattttttgacacttcatttttataattatcaagaaattattaattttataattattaaaagctaccagtgtcttcaggctttgcatctctagcacaaggggtatcattattcccgagtggcacatcttcattcccaattcagaaagtacacattgccctgcacgtctcccacggcaagctgcagggtggagttagcgcccagccaaggttccaggcagctcactgacccttcgcatcggaacaggcccagcagctgcatactgggtctctcccatagcttaacatctctgtccttcgaagctgtcaccagcaactcaggtagcacatggagggctgtgacagagcccgagtgaatctttctacgctgccgtgtctttagatgtggtgttggctcactatccatgctggcatcactatccatgctggcatcagattccctgcaggtagatgggtctgtccctggagtttgggtttctggagtgtttgcttttttctgccacatgttacctgtggtccattctccttctgggctgcatttggccaggttccataggatcccatcagagctggcacacaaaaatgaggactcagattcaggtttggcttgagttatcgatattagggtcctactaggattctctaagtttatatcaaagttcagcctctcttcaaactctcctgattccttttgcctcaagaaagaaagaactccaggatccttgggctgcaggacaaatatgccatactccttgtgggtggacaatatcataggattttctgtatagctgctccagatttcagatggagcatcccctggcttcatgcaaagtaacttcaaatctgctttggccaagatgagaaagtgaccatcaggagcccaatccagacttgtcagcacccctaagtcctcctgtagaattcggttcaggtgaagactcaaatttccgggtgccgaacccttccgcagtttcacttgccactcgctgattttctcatcagcactgaggacaaaaaaggtgtgtgccgaggaccagatcagagcaccaatgtggcctggagcctgtgctgtggccacagccttagcttcctgccacaagattagttccccagcttgatttccagatactgccatggaaccatctggtgcccaagccacagcagtgacggctgcagaactccttggtatacatgtgtcatctgcttccttaggaacctgccagagccgtacagaaccatcctcagaggcggtcagcatgaggcctgaggtttctgaaacagcagcagcacggactgggccgctgtgtcccaggagggtgtgggtttggcacaccaagagtggatgccataaccgtgtggccccatctagcccgacggttaccaccagaagctctgacccaggctgtccagctgcacggggctccatggcagctgcacagtggctaatgggtcctgagtgagcagggatgctggtcagctccacgccttgatggtcccacactttcaaggtcccatcccggctcacagacaccacgtgctcctccacagctgccacagcgctcacagcactctgatgacccaggaactgaccaagccgctgtcctgactctgggtcccagagccccacagagccatcactggagcaggatatcagtaggttatctttggtccaggcacagccagtgacccagtcacggtgacaggcagggaaggagtggatcaaaacaggggttttgggtgtcctcacgtcccagcagaggagactccgatcccggcccccggtggccaggctgcctccatcagtgctgaaactacagcagctcacagggccctcatgtccccgcagctcagtgccacagggaaagtcttctgccttgtgtggccgcgtcagcagctgccttggccacagctgcactgtgaaatcctctgaggcagaagccaagagctcctgggaagtggccagtcctagcacaggcttctggaatctggacaggagccagagggactgaagggagcattccttgagtgcccagccctgcaaggacccatcttctgcaccactcaccaataccttggggcttagccaggccagggcggacactgccacatccagtgcctgaccctgagccccctgggaacctgaagagattttgtagatcctaatgccatccgctcgatatccaacagccacccgatcaccatctgggctgagtgccacagagagggcaggagagagagaaagggaacccaggtgcccacggggccgacccagagaccctgaccacacctgaaccttgccatcctctccagccgtcagtaactggcaacccgcatgcaggaaaagcgcagcagcaacaaagccatggtgggcagggaaggcagccagccgtgccccttctcgccaggcccacagctccaccatactgtccagccggcccacagccacaacccccccaggcacattgaaggccaaggtacggatagaggctccgggtgcccccaggtccttggtgactttgagcccatccacctggaagaagctgatgctgccagcccagctgcctgtggctattacctgcccctctgggtggaaggcaacacagttcagggacttggggtaggtgtgctggaaggccagctgcccacggactgtgtcccacagctttaggcatcctcccaagcacacggtggctagcagccggcagtctgggctcaggcagcagccagtgatttggtactggtgagccttagtctgcagcacccgacaaccatgctgcaggtcccagagctccaggagcccgtcgaaggcagtaagaaagagtgtatcatcggagaggaacaaacaagcagagattccatcacagccactcaccacagacttctcctcctgccaagttctcaggtccaacaggtaaactgtcccattggcagtgcccacagctgctctttgcccattggtggagaaggccacagcagtaggggatgaggaaactgccagagacaggctggagctttgctgatttttcatggtccggggtttattaagccatcgtagtgtgtgttggaggtgccatctccgggagagcagcgaggcttggtggcaaagaggtgagtccaggggctggttggctgcctgctggggcaggagccgggggtactggctgaggattgaagcctgctgcctcaggaaggtgcgaaacactgcaacgtcagcctcggggagcttttgttcctctttggggactgaagaagcatagagggcatgggcctccaagagccgagagaccagacccaattccaagtgtgcagccaccacatggaggttggtaaggaacttcgaaagaagtccacggttcccgctctggagcaggtggtaaggcaggtctcccagagcctcaggagggcaacttcggaaggtgcctgaggcatcagcgtcacatgtcttccagagctgagctgcaatgaggatgtgtgccgtgtcctctagccctggcctcttcccatagcaacgtttagctgctgttctcaggggcccatcagggaggcacagccgggcaccagggcgctccagagggccctcccctagcaaactgcgcagactctggacgaggcaggcaaacgggcccatggggtaggggtctccactgttaccagcagccactgcttcttcccagctcttagtccccttcggtagtgtccgccacacactcagcactccgtgcagctggtccacagtcaaaccactccgtgtgacttctagggcagtcaaggcctggggaaggacatcaggcccgtgctccttctccagtgtgctcaggatgtgctgcagcagcagggggacagtggcaggcagggtccggagtctctcagacacctgctcatacagcgtgaagagcctcaggtgatcggtgaccaagcgcaggtagagcggccggcctgattcccgcttcaccagcagcagtcgcatctggttgttaaatggtgactcctccagccgcttcccgtacagggccagctcctctctcaccagccgggcccgagcagaggcctccagaggccccaaggccagcacgtgggcaccctggctctgctcaagggtctcccctaggcctgcatcactagacacactcagcaccaggtgtacacaccggggaagcttctttgggatccagtctgaaatcagctgcccattctggtccactaacctatcagccccatcgatgatcaggacctgggtctggccaggatgcagggactcagcagacttgggcagcagcctctgctgcagctcccacaccaggcttcggtaggtgctggggagggcacctggctcttttagttggccacgcagataggtacagaggcgtctgagcagagtgagggcaagaccctggtcaggacgagccccagaaaagtggaagaagactaatgatgccaccttggccccatcaggagcctgcagggctgacacaagagatgccaggaaggctgtcttgccctgtcctgactgccccgtcaccaggctcagccttccgtggggcagcatcagccgttgcactgtgtcctgaagaaggcgtggccgggcaggactcggtggcttctgcagctgctggaaggtggcctggaccaagtcatcgtctgggatggacactggctgctccagcagggccccaggctgcaggtagagcttctggatcatattccatacatcctgcagaaccaactgcccaaactcctccagcccgccaacatagggccggccagctgccacacccccccactcacaggggtatctgcggcaggtgatccctttctgtctgcttaggtagctcttcagttctgagatccgacgtgcggcctcttcagactcagaaacaaagtcagatttccaggcatctggcacagagctgaggaagctggaatcccggaagtagatgagagcttgggcagagggctgcagacgttggttccggttcaggaactgcatcacctccatctctgtcacagagcgccctgaagggtactgctgggcccagtggaagtgtggatggtcaggaaggttgtagctggggggaatgtatccataacgggagcccagaatccccacaaacagctgtgcgttctccacctccccaaggcacacttccagttgtctgttcctacgggtctcctcctcagtgacgccccagcggaggtcgattccgtgaaggctgatacggtgaggggccgctcgggcctgcagtgctggcagcacagacctcagcagcaggtcccgctccccatgcatgtctcggaaagtggatgaaatgaaaagccggatgctgcgccatccttgctgggaaacaggagccaaggggcttggagtgtcctcttccagtggccggagagactggacccctgtctttcctgggggtggtggaatcttgaatattttgtccatttggcccacatgttccagaagatgggaggccccatgctctgcaatgaacttcagtatcgcatcagtacagcctgagagtgtcacatcattgggattcaaatctgttgacaggtattgtacccttcttaggaggataccaacaaagaggcacttggaattcacacgctgccagtaaagctgtttggccacatttatcattccatcatccatgctttggccaaggaggatgaccctgtccacaggaaccctttggccagccagagacagcaggtatttcccaaaagtattcagggaccatccatcattttcatcaaactcctggacttgagcctggagcttgatggcagtcttcaggatgccttcttctgccttaagcactgcagtcttcagagtgtcacctccacacagcacgacgtccacctgctccgccctcgtgatcatcatcccaatcaacagcagtgcatagttcagcgggggcccttgtgggttgctctttggacagagcctgtctgcattagcatctgtcagatagaccaagacagtgcggcctggcagcaggggcaggctgtgcttcacagagaggttcacagctgtctctagggcctgtcggtacctgttcagcatctcaccatcatatttccactgtctggccttgtgtactctcagcttctccctcttgagctgctcatacaacacaggtatcctcattgccatccgaagctgctgacggcttaggtggcaaagaaacctccgcctgggacggttcttttcatttctagttagtatccgcctcatcagtgttatattcgaaggaaagggcaatgcttgatttctgagttgagcctcgagggcatcaatggcatcatgggcgttaagaaatctgaatggaaactgccgactgtggatcaccgacttcgcatgctggagtctctggagaatgagctcatggtggcgggaactgattccaacccgcagcaggttgcacaggttccgaagcatggccatgaagggaagcttcccattttcaatgagttcctcccagaccgacgctttgttcccccgtaggctcagctcccgctcccaggtctctggcctagacagcttcatcctcttcccagctctgctagaatcccaaggcccaggaaggcgacttcgagaaaagagctgtaggttggaggggtatctgtaacccagcagggcttgaacgtgctgggcaggcttgtggatgtgcagtcgctgaaccagcttcttcagggtgaaccttggaggattctttttctctgacactgtatcaccggccttctcaaactttctctgctcttctctgagaaaccctatgtaccttggaaaacatctgtgagaaaatggaggctccatccccttgaggataaactcaggctccaggagggcaagttcacgacagatttcaaaaatggcagccagggtggggtcagatgtattgttcatgtttacttctgagaccagagtagagcacagcaagctcagtagagccatcttcttttcctgaaggacatggtcagtaggctctggatgagattcagagtctccagaggtgagcttcacggccagatcctccacctcctcctcctctcccaagctcagactataagaaggcatttgggtctctgcccctttcttctcttctgaatcaaaccaacgacccaaagttgcttcctgagctgtctctgtggcagagatggatttcagggctatagggcaggttgaaaggtctagtcccttagagaaatgctgagccctccaacttggaggctcagagagcaggcaattgctgttgttcacacggtacaaatcagcttgcgtcatgtgagatatctgtagactctggaacaaggggctggcagacacagtgctctttagactagagagggtggccaggcaccggttctccaaggagaggatgtctgggtgggcagaaacatgtccatgtggtttctccatggtcttcaggtcagaaagtgtggccaggcactggttctccaaggagaggatgtctgggtgggcagacacatatccatgtggtttttccatggtcttcaggtcaggaagcgtggctaggcactggttcttcaaggagaggatatctgagtgggtagatacatgctgatgtagtttctccaagggctgtaagtcagggagcatagccaggcaccggttctccaaggagaggatgtctggatgggcagacacatgcccatggagtttttccatggctgaaactcagcttgtatatgcctggggcgtccgattcccgcagcaggaagcagaaacttcgctctggattctgccggtgggaagggtggcagccgggggaggagccggatgcggatct

SEQ ID NO: 11393 - RNA, 8710 nt, Homo sapiens
  source 1..8710: mol_type = other RNA
ctgaatagctgggactacaggtgcccgccgccacacctggctaactttttgtattttttagtagagacagggtttcactatgttagccaggatggtcttgatctcctgacctcgtgatctgcccacctcggcctcccaaagtgctgggattacaagcgtgagccaccatgcccggcctcctctgggtagttctgagaaaagggctgtctctgtgacagaaacatagctctttctaaatgccctgatgcatgactgacttattctccctccctcattctttcccgatgaactgaaaggtcttccatgctctgttcaaattgaatgttggccaacatcactctcattcctcctcctggcaagaatggcatcctagggtcctagggcccgcgagtgatgcaagaattctaaaacctagtttcaaaagagtacctactaaagatttcattcactttcttgtggttctagtaaggattaatgttgaataagaagagacacacattagaatgtacatatacatacacatagaatatcctcctgttctaaatccacatgagaacacaggcaggcctacacttgagattttttgacacttcatttttataattatcaagaaattattaattttataattattaaaagctaccagtgtcttcaggctttgcatctctagcacaaggggtatcattattcccgagtggcacatcttcattcccaattcagaaagtacacattgccctgcacgtctcccacggcaagctgcagggtggagttagcgcccagccaaggttccaggcagctcactgacccttcgcatcggaacaggcccagcagctgcatactgggtctctcccatagcttaacatctctgtccttcgaagctgtcaccagcaactcaggtagcacatggagggctgtgacagagcccgagtgaatctttctacgctgccgtgtctttagatgtggtgttggctcactatccatgctggcatcactatccatgctggcatcagattccctgcaggtagatgggtctgtccctggagtttgggtttctggagtgtttgcttttttctgccacatgttacctgtggtccattctccttctgggctgcatttggccaggttccataggatcccatcagagctggcacacaaaaatgaggactcagattcaggtttggcttgagttatcgatattagggtcctactaggattctctaagtttatatcaaagttcagcctctcttcaaactctcctgattccttttgcctcaagaaagaaagaactccaggatccttgggctgcaggacaaatatgccatactccttgtgggtggacaatatcataggattttctgtatagctgctccagatttcagatggagcatcccctggcttcatgcaaagtaacttcaaatctgctttggccaagatgagaaagtgaccatcaggagcccaatccagacttgtcagcacccctaagtcctcctgtagaattcggttcaggtgaagactcaaatttccgggtgccgaacccttccgcagtttcacttgccactcgctgattttctcatcagcactgaggacaaaaaaggtgtgtgccgaggaccagatcagagcaccaatgtggcctggagcctgtgctgtggccacagccttagcttcctgccacaagattagttccccagcttgatttccagatactgccatggaaccatctggtgcccaagccacagcagtgacggctgcagaactccttggtatacatgtgtcatctgcttccttaggaacctgccagagccgtacagaaccatcctcagaggcggtcagcatgaggcctgaggtttctgaaacagcagcagcacggactgggccgctgtgtcccaggagggtgtgggtttggcacaccaagagtggatgccataaccgtgtggccccatctagcccgacggttaccaccagaagctctgacccaggctgtccagctgcacggggctccatggcagctgcacagtggctaatgggtcctgagtgagcagggatgctggtcagctccacgccttgatggtcccacactttcaaggtcccatcccggctcacagacaccacgtgctcctccacagctgccacagcgctcacagcactctgatgacccaggaactgaccaagccgctgtcctgactctgggtcccagagccccacagagccatcactggagcaggatatcagtaggttatctttggtccaggcacagccagtgacccagtcacggtgacaggcagggaaggagtggatcaaaacaggggttttgggtgtcctcacgtcccagcagaggagactccgatcccggcccccggtggccaggctgcctccatcagtgctgaaactacagcagctcacagggccctcatgtccccgcagctcagtgccacagggaaagtcttctgccttgtgtggccgcgtcagcagctgccttggccacagctgcactgtgaaatcctctgaggcagaagccaagagctcctgggaagtggccagtcctagcacaggcttctggaatctggacaggagccagagggactgaagggagcattccttgagtgcccagccctgcaaggacccatcttctgcaccactcaccaataccttggggcttagccaggccagggcggacactgccacatccagtgcctgaccctgagccccctgggaacctgaagagattttgtagatcctaatgccatccgctcgatatccaacagccacccgatcaccatctgggctgagtgccacagagagggcaggagagagagaaagggaacccaggtgcccacggggccgacccagagaccctgaccacacctgaaccttgccatcctctccagccgtcagtaactggcaacccgcatgcaggaaaagcgcagcagcaacaaagccatggtgggcagggaaggcagccagccgtgccccttctcgccaggcccacagctccaccatactgtccagccggcccacagccacaacccccccaggcacattgaaggccaaggtacggatagaggctccgggtgcccccaggtccttggtgactttgagcccatccacctggaagaagctgatgctgccagcccagctgcctgtggctattacctgcccctctgggtggaaggcaacacagttcagggacttggggtaggtgtgctggaaggccagctgcccacggactgtgtcccacagctttaggcatcctcccaagcacacggtggctagcagccggcagtctgggctcaggcagcagccagtgatttggtactggtgagccttagtctgcagcacccgacaaccatgctgcaggtcccagagctccaggagcccgtcgaaggcagtaagaaagagtgtatcatcggagaggaacaaacaagcagagattccatcacagccactcaccacagacttctcctcctgccaagttctcaggtccaacaggtaaactgtcccattggcagtgcccacagctgctctttgcccattggtggagaaggccacagcagtaggggatgaggaaactgccagagacaggctggagctttgctgatttttcatggtccggggtttattaagccatcgtagtgtgtgttggaggtgccatctccgggagagcagcgaggcttggtggcaaagaggtgagtccaggggctggttggctgcctgctggggcaggagccgggggtactggctgaggattgaagcctgctgcctcaggaaggtgcgaaacactgcaacgtcagcctcggggagcttttgttcctctttggggactgaagaagcatagagggcatgggcctccaagagccgagagaccagacccaattccaagtgtgcagccaccacatggaggttggtaaggaacttcgaaagaagtccacggttcccgctctggagcaggtggtaaggcaggtctcccagagcctcaggagggcaacttcggaaggtgcctgaggcatcagcgtcacatgtcttccagagctgagctgcaatgaggatgtgtgccgtgtcctctagccctggcctcttcccatagcaacgtttagctgctgttctcaggggcccatcagggaggcacagccgggcaccagggcgctccagagggccctcccctagcaaactgcgcagactctggacgaggcaggcaaacgggcccatggggtaggggtctccactgttaccagcagccactgcttcttcccagctcttagtccccttcggtagtgtccgccacacactcagcactccgtgcagctggtccacagtcaaaccactccgtgtgacttctagggcagtcaaggcctggggaaggacatcaggcccgtgctccttctccagtgtgctcaggatgtgctgcagcagcagggggacagtggcaggcagggtccggagtctctcagacacctgctcatacagcgtgaagagcctcaggtgatcggtgaccaagcgcaggtagagcggccggcctgattcccgcttcaccagcagcagtcgcatctggttgttaaatggtgactcctccagccgcttcccgtacagggccagctcctctctcaccagccgggcccgagcagaggcctccagaggccccaaggccagcacgtgggcaccctggctctgctcaagggtctcccctaggcctgcatcactagacacactcagcaccaggtgtacacaccggggaagcttctttgggatccagtctgaaatcagctgcccattctggtccactaacctatcagccccatcgatgatcaggacctgggtctggccaggatgcagggactcagcagacttgggcagcagcctctgctgcagctcccacaccaggcttcggtaggtgctggggagggcacctggctcttttagttggccacgcagataggtacagaggcgtctgagcagagtgagggcaagaccctggtcaggacgagccccagaaaagtggaagaagactaatgatgccaccttggccccatcaggagcctgcagggctgacacaagagatgccaggaaggctgtcttgccctgtcctgactgccccgtcaccaggctcagccttccgtggggcagcatcagccgttgcactgtgtcctgaagaaggcgtggccgggcaggactcggtggcttctgcagctgctggaaggtggcctggaccaagtcatcgtctgggatggacactggctgctccagcagggccccaggctgcaggtagagcttctggatcatattccatacatcctgcagaaccaactgcccaaactcctccagcccgccaacatagggccggccagctgccacacccccccactcacaggggtatctgcggcaggtgatccctttctgtctgcttaggtagctcttcagttctgagatccgacgtgcggcctcttcagactcagaaacaaagtcagatttccaggcatctggcacagagctgaggaagctggaatcccggaagtagatgagagcttgggcagagggctgcagacgttggttccggttcaggaactgcatcacctccatctctgtcacagagcgccctgaagggtactgctgggcccagtggaagtgtggatggtcaggaaggttgtagctggggggaatgtatccataacgggagcccagaatccccacaaacagctgtgcgttctccacctccccaaggcacacttccagttgtctgttcctacgggtctcctcctcagtgacgccccagcggaggtcgattccgtgaaggctgatacggtgaggggccgctcgggcctgcagtgctggcagcacagacctcagcagcaggtcccgctccccatgcatgtctcggaaagtggatgaaatgaaaagccggatgctgcgccatccttgctgggaaacaggagccaaggggcttggagtgtcctcttccagtggccggagagactggacccctgtctttcctgggggtggtggaatcttgaatattttgtccatttggcccacatgttccagaagatgggaggccccatgctctgcaatgaacttcagtatcgcatcagtacagcctgagagtgtcacatcattgggattcaaatctgttgacaggtattgtacccttcttaggaggataccaacaaagaggcacttggaattcacacgctgccagtaaagctgtttggccacatttatcattccatcatccatgctttggccaaggaggatgaccctgtccacaggaaccctttggccagccagagacagcaggtatttcccaaaagtattcagggaccatccatcattttcatcaaactcctggacttgagcctggagcttgatggcagtcttcaggatgccttcttctgccttaagcactgcagtcttcagagtgtcacctccacacagcacgacgtccacctgctccgccctcgtgatcatcatcccaatcaacagcagtgcatagttcagcgggggcccttgtgggttgctctttggacagagcctgtctgcattagcatctgtcagatagaccaagacagtgcggcctggcagcaggggcaggctgtgcttcacagagaggttcacagctgtctctagggcctgtcggtacctgttcagcatctcaccatcatatttccactgtctggccttgtgtactctcagcttctccctcttgagctgctcatacaacacaggtatcctcattgccatccgaagctgctgacggcttaggtggcaaagaaacctccgcctgggacggttcttttcatttctagttagtatccgcctcatcagtgttatattcgaaggaaagggcaatgcttgatttctgagttgagcctcgagggcatcaatggcatcatgggcgttaagaaatctgaatggaaactgccgactgtggatcaccgacttcgcatgctggagtctctggagaatgagctcatggtggcgggaactgattccaacccgcagcaggttgcacaggttccgaagcatggccatgaagggaagcttcccattttcaatgagttcctcccagaccgacgctttgttcccccgtaggctcagctcccgctcccaggtctctggcctagacagcttcatcctcttcccagctctgctagaatcccaaggcccaggaaggcgacttcgagaaaagagctgtaggttggaggggtatctgtaacccagcagggcttgaacgtgctgggcaggcttgtggatgtgcagtcgctgaaccagcttcttcagggtgaaccttggaggattctttttctctgacactgtatcaccggccttctcaaactttctctgctcttctctgagaaaccctatgtaccttggaaaacatctgtgagaaaatggaggctccatccctggagagcggggtggccggcgggggtgtctcttggcccggtgcttccgagggttgtacttagccagctggtactcgtcaaactgggcaaatttgtccgtcatggcagtacggagacaggcgggcaggggcaccagcttattcttatctccctcagccaggctctggtaaagctcagccacctggatccagtcagaaggcagctggacaatggcacagaaatatcgtcgcaggtgggggcgacacgccggcaagaaagcagcaatggccaagatgttattggccacattccggacgttcagctgctgcctggcatacaaagatgccttgaggataaactcaggctccaggagggcaagttcacgacagatttcaaaaatggcagccagggtggggtcagatgtattgttcatgtttacttctgagaccagagtagagcacagcaagctcagtagagccatcttcttttcctgaaggacatggtcagtaggctctggatgagattcagagtctccagaggtgagcttcacggccagatcctccacctcctcctcctctcccaagctcagactataagaaggcatttgggtctctgcccctttcttctcttctgaatcaaaccaacgacccaaagttgcttcctgagctgtctctgtggcagagatggatttcagggctatagggcaggttgaaaggtctagtcccttagagaaatgctgagccctccaacttggaggctcagagagcaggcaattgctgttgttcacacggtacaaatcagcttgcgtcatgtgagatatctgtagactctggaacaaggggctggcagacacagtgctctttagactagagagggtggccaggcaccggttctccaaggagaggatgtctgggtgggcagaaacatgtccatgtggtttctccatggtcttcaggtcagaaagtgtggccaggcactggttctccaaggagaggatgtctgggtgggcagacacatatccatgtggtttttccatggtcttcaggtcaggaagcgtggctaggcactggttcttcaaggagaggatatctgagtgggtagatacatgctgatgtagtttctccaagggctgtaagtcagggagcatagccaggcaccggttctccaaggagaggatgtctggatgggcagacacatgcccatggagtttttccatggctgaaactcagcttgtatatgcctggggcgtccgattcccgcagcaggaagcagaaacttcgctctggattctgccggtgggaagggtggcagccgggggaggagccggatgcggatct

SEQ ID NO: 11394 - RNA, 8768 nt, Homo sapiens
  source 1..8768: mol_type = other RNA
ctgaatagctgggactacaggtgcccgccgccacacctggctaactttttgtattttttagtagagacagggtttcactatgttagccaggatggtcttgatctcctgacctcgtgatctgcccacctcggcctcccaaagtgctgggattacaagcgtgagccaccatgcccggcctcctctgggtagttctgagaaaagggctgtctctgtgacagaaacatagctctttctaaatgccctgatgcatgactgacttattctccctccctcattctttcccgatgaactgaaaggtcttccatgctctgttcaaattgaatgttggccaacatcactctcattcctcctcctggcaagaatggcatcctagggtcctagggcccgcgagtgatgcaagaattctaaaacctagtttcaaaagagtacctactaaagatttcattcactttcttgtggttctagtaaggattaatgttgaataagaagagacacacattagaatgtacatatacatacacatagaatatcctcctgttctaaatccacatgagaacacaggcaggcctacacttgagattttttgacacttcatttttataattatcaagaaattattaattttataattattaaaagctaccagtgtcttcaggctttgcatctctagcacaaggggtatcattattcccgagtggcacatcttcattcccaattcagaaagtacacattgccctgcacgtctcccacggcaagctgcagggtggagttagcgcccagccaaggttccaggcagctcactgacccttcgcatcggaacaggcccagcagctgcatactgggtctctcccatagcttaacatctctgtccttcgaagctgtcaccagcaactcaggtagcacatggagggctgtgacagagcccgagtgaatctttctacgctgccgtgtctttagatgtggtgttggctcactatccatgctggcatcactatccatgctggcatcagattccctgcaggtagatgggtctgtccctggagtttgggtttctggagtgtttgcttttttctgccacatgttacctgtggtccattctccttctgggctgcatttggccaggttccataggatcccatcagagctggcacacaaaaatgaggactcagattcaggtttggcttgagttatcgatattagggtcctactaggattctctaagtttatatcaaagttcagcctctcttcaaactctcctgattccttttgcctcaagaaagaaagaactccaggatccttgggctgcaggacaaatatgccatactccttgtgggtggacaatatcataggattttctgtatagctgctccagatttcagatggagcatcccctggcttcatgcaaagtaacttcaaatctgctttggccaagatgagaaagtgaccatcaggagcccaatccagacttgtcagcacccctaagtcctcctgtagaattcggttcaggtgaagactcaaatttccgggtgccgaacccttccgcagtttcacttgccactcgctgattttctcatcagcactgaggacaaaaaaggtgtgtgccgaggaccagatcagagcaccaatgtggcctggagcctgtgctgtggccacagccttagcttcctgccacaagattagttccccagcttgatttccagatactgccatggaaccatctggtgcccaagccacagcagtgacggctgcagaactccttggtatacatgtgtcatctgcttccttaggaacctgccagagccgtacagaaccatcctcagaggcggtcagcatgaggcctgaggtttctgaaacagcagcagcacggactgggccgctgtgtcccaggagggtgtgggtttggcacaccaagagtggatgccataaccgtgtggccccatctagcccgacggttaccaccagaagctctgacccaggctgtccagctgcacggggctccatggcagctgcacagtggctaatgggtcctgagtgagcagggatgctggtcagctccacgccttgatggtcccacactttcaaggtcccatcccggctcacagacaccacgtgctcctccacagctgccacagcgctcacagcactctgatgacccaggaactgaccaagccgctgtcctgactctgggtcccagagccccacagagccatcactggagcaggatatcagtaggttatctttggtccaggcacagccagtgacccagtcacggtgacaggcagggaaggagtggatcaaaacaggggttttgggtgtcctcacgtcccagcagaggagactccgatcccggcccccggtggccaggctgcctccatcagtgctgaaactacagcagctcacagggccctcatgtccccgcagctcagtgccacagggaaagtcttctgccttgtgtggccgcgtcagcagctgccttggccacagctgcactgtgaaatcctctgaggcagaagccaagagctcctgggaagtggccagtcctagcacaggcttctggaatctggacaggagccagagggactgaagggagcattccttgagtgcccagccctgcaaggacccatcttctgcaccactcaccaataccttggggcttagccaggccagggcggacactgccacatccagtgcctgaccctgagccccctgggaacctgaagagattttgtagatcctaatgccatccgctcgatatccaacagccacccgatcaccatctgggctgagtgccacagagagggcaggagagagagaaagggaacccaggtgcccacggggccgacccagagaccctgaccacacctgaaccttgccatcctctccagccgtcagtaactggcaacccgcatgcaggaaaagcgcagcagcaacaaagccatggtgggcagggaaggcagccagccgtgccccttctcgccaggcccacagctccaccatactgtccagccggcccacagccacaacccccccaggcacattgaaggccaaggtacggatagaggctccgggtgcccccaggtccttggtgactttgagcccatccacctggaagaagctgatgctgccagcccagctgcctgtggctattacctgcccctctgggtggaaggcaacacagttcagggacttggggtaggtgtgctggaaggccagctgcccacggactgtgtcccacagctttaggcatcctcccaagcacacggtggctagcagccggcagtctgggctcaggcagcagccagtgatttggtactggtgagccttagtctgcagcacccgacaaccatgctgcaggtcccagagctccaggagcccgtcgaaggcagtaagaaagagtgtatcatcggagaggaacaaacaagcagagattccatcacagccactcaccacagacttctcctcctgccaagttctcaggtccaacaggtaaactgtcccattggcagtgcccacagctgctctttgcccattggtggagaaggccacagcagtaggggatgaggaaactgccagagacaggctggagctttgctgatttttcatggtccggggtttattaagccatcgtagtgtgtgttggaggtgccatctccgggagagcagcgaggcttggtggcaaagaggtgagtccaggggctggttggctgcctgctggggcaggagccgggggtactggctgaggattgaagcctgctgcctcaggaaggtgcgaaacactgcaacgtcagcctcggggagcttttgttcctctttggggactgaagaagcatagagggcatgggcctccaagagccgagagaccagacccaattccaagtgtgcagccaccacatggaggttggtaaggaacttcgaaagaagtccacggttcccgctctggagcaggtggtaaggcaggtctcccagagcctcaggagggcaacttcggaaggtgcctgaggcatcagcgtcacatgtcttccagagctgagctgcaatgaggatgtgtgccgtgtcctctagccctggcctcttcccatagcaacgtttagctgctgttctcaggggcccatcagggaggcacagccgggcaccagggcgctccagagggccctcccctagcaaactgcgcagactctggacgaggcaggcaaacgggcccatggggtaggggtctccactgttaccagcagccactgcttcttcccagctcttagtccccttcggtagtgtccgccacacactcagcactccgtgcagctggtccacagtcaaaccactccgtgtgacttctagggcagtcaaggcctggggaaggacatcaggcccgtgctccttctccagtgtgctcaggatgtgctgcagcagcagggggacagtggcaggcagggtccggagtctctcagacacctgctcatacagcgtgaagagcctcaggtgatcggtgaccaagcgcaggtagagcggccggcctgattcccgcttcaccagcagcagtcgcatctggttgttaaatggtgactcctccagccgcttcccgtacagggccagctcctctctcaccagccgggcccgagcagaggcctccagaggccccaaggccagcacgtgggcaccctggctctgctcaagggtctcccctaggcctgcatcactagacacactcagcaccaggtgtacacaccggggaagcttctttgggatccagtctgaaatcagctgcccattctggtccactaacctatcagccccatcgatgatcaggacctgggtctggccaggatgcagggactcagcagacttgggcagcagcctctgctgcagctcccacaccaggcttcggtaggtgctggggagggcacctggctcttttagttggccacgcagataggtacagaggcgtctgagcagagtgagggcaagaccctggtcaggacgagccccagaaaagtggaagaagactaatgatgccaccttggccccatcaggagcctgcagggctgacacaagagatgccaggaaggctgtcttgccctgtcctgactgccccgtcaccaggctcagccttccgtggggcagcatcagccgttgcactgtgtcctgaagaaggcgtggccgggcaggactcggtggcttctgcagctgctggaaggtggcctggaccaagtcatcgtctgggatggacactggctgctccagcagggccccaggctgcaggtagagcttctggatcatattccatacatcctgcagaaccaactgcccaaactcctccagcccgccaacatagggccggccagctgccacacccccccactcacaggggtatctgcggcaggtgatccctttctgtctgcttaggtagctcttcagttctgagatccgacgtgcggcctcttcagactcagaaacaaagtcagatttccaggcatctggcacagagctgaggaagctggaatcccggaagtagatgagagcttgggcagagggctgcagacgttggttccggttcaggaactgcatcacctccatctctgtcacagagcgccctgaagggtactgctgggcccagtggaagtgtggatggtcaggaaggttgtagctggggggaatgtatccataacgggagcccagaatccccacaaacagctgtgcgttctccacctccccaaggcacacttccagttgtctgttcctacgggtctcctcctcagtgacgccccagcggaggtcgattccgtgaaggctgatacggtgaggggccgctcgggcctgcagtgctggcagcacagacctcagcagcaggtcccgctccccatgcatgtctcggaaagtggatgaaatgaaaagccggatgctgcgccatccttgctgggaaacaggagccaaggggcttggagtgtcctcttccagtggccggagagactggacccctgtctttcctgggggtggtggaatcttgaatattttgtccatttggcccacatgttccagaagatgggaggccccatgctctgcaatgaacttcagtatcgcatcagtacagcctgagagtgtcacatcattgggattcaaatctgttgacaggtattgtacccttcttaggaggataccaacaaagaggcacttggaattcacacgctgccagtaaagctgtttggccacatttatcattccatcatccatgctttggccaaggaggatgaccctgtccacaggaaccctttggccagccagagacagcaggtatttcccaaaagtattcagggaccatccatcattttcatcaaactcctggacttgagcctggagcttgatggcagtcttcaggatgccttcttctgccttaagcactgcagtcttcagagtgtcacctccacacagcacgacgtccacctgctccgccctcgtgatcatcatcccaatcaacagcagtgcatagttcagcgggggcccttgtgggttgctctttggacagagcctgtctgcattagcatctgtcagatagaccaagacagtgcggcctggcagcaggggcaggctgtgcttcacagagaggttcacagctgtctctagggcctgtcggtacctgttcagcatctcaccatcatatttccactgtctggccttgtgtactctcagcttctccctcttgagctgctcatacaacacaggtatcctcattgccatccgaagctgctgacggcttaggtggcaaagaaacctccgcctgggacggttcttttcatttctagttagtatccgcctcatcagtgttatattcgaaggaaagggcaatgcttgatttctgagttgagcctcgagggcatcaatggcatcatgggcgttaagaaatctgaatggaaactgccgactgtggatcaccgacttcgcatgctggagtctctggagaatgagctcatggtggcgggaactgattccaacccgcagcaggttgcacaggttccgaagcatggccatgaagggaagcttcccattttcaatgagttcctcccagaccgacgctttgttcccccgtaggctcagctcccgctcccaggtctctggcctagacagcttcatcctcttcccagctctgctagaatcccaaggcccaggaaggcgacttcgagaaaagagctgtaggttggaggggtatctgtaacccagcagggcttgaacgtgctgggcaggcttgtggatgtgcagtcgctgaaccagcttcttcagggtgaaccttggaggattctttttctctgacactgtatcaccggccttctcaaactttctctgctcttctctgagaaaccctatgtaccttggaaaacatctgtgagaaaatggaggctccatccctggagagcggggtggccggcgggggtgtctcttggcccggtgcttccgagggttgtacttagccagctggtactcgtcaaactgggcaaatttgtccgtcatggcagtacggagacaggcgggcaggggcaccagcttattcttatctccctcagccaggctctggtaaagctcagccacctggatccagtcagaaggcagctggacaatggcacagaaatatcgtcgcaggtgggggcgacacgccggcaagaaagcagcaatggccaagatgttattggccacattccggacgttcagctgctgcctggcatacaaagatgccttgaggataaactcaggctccaggagggcaagttcacgacagatttcaaaaatggcagccagggtggggtcagatgtattgttcatgtttacttctgagaccagagtagagcacagcaagctcagtagagccatcttcttttcctgaaggacatggtcagtaggctctggatgagattcagagtctccagaggtgagcttcacggccagatcctccacctcctcctcctctcccaagctcagactataagaaggcatttgggtctctgcccctttcttctcttctgaatcaaaccaacgacccaaagttgcttcctgagctgtctctgtggcagagatggatttcagggctatagggcaggttgaaaggtctagtcccttagagaaatgctgagccctccaacttggaggctcagagagcaggcaattgctgttgttcacacggtacaaatcagcttgcgtcatgtgagatatctgtagactctggaacaaggggctggcagacacagtgctctttagactagagagggtggccaggcaccggttctccaaggagaggatgtctgggtgggcagaaacatgtccatgtggtttctccatggtcttcaggtcagaaagtgtggccaggcactggttctccaaggagaggatgtctgggtgggcagacacatatccatgtggtttttccatggtcttcaggtcaggaagcgtggctaggcactggttcttcaaggagaggatatctgagtgggtagatacatgctgatgtagtttctccaagggctgtaagtcagggagcatagccaggcaccggttctccaaggagaggatgtctggatgggcagacacatgcccatggagtttttccatggctgaaactcagcttgtatatgccttagactggggctggaaaccctgggtgcctgacctggggcgtccgattcccgcagcaggaagcagaaacttcgctctggattctgccggtgggaagggtggcagccgggggaggagccggatgcggatctgagaagagacggtgcgggcggaga

SEQ ID NO: 11395 - RNA, 7114 nt, Homo sapiens
  source 1..7114: mol_type = other RNA
ctgaatagctgggactacaggtgcccgccgccacacctggctaactttttgtattttttagtagagacagggtttcactatgttagccaggatggtcttgatctcctgacctcgtgatctgcccacctcggcctcccaaagtgctgggattacaagcgtgagccaccatgcccggcctcctctgggtagttctgagaaaagggctgtctctgtgacagaaacatagctctttctaaatgccctgatgcatgactgacttattctccctccctcattctttcccgatgaactgaaaggtcttccatgctctgttcaaattgaatgttggccaacatcactctcattcctcctcctggcaagaatggcatcctagggtcctagggcccgcgagtgatgcaagaattctaaaacctagtttcaaaagagtacctactaaagatttcattcactttcttgtggttctagtaaggattaatgttgaataagaagagacacacattagaatgtacatatacatacacatagaatatcctcctgttctaaatccacatgagaacacaggcaggcctacacttgagattttttgacacttcatttttataattatcaagaaattattaattttataattattaaaagctaccagtgtcttcaggctttgcatctctagcacaaggggtatcattattcccgagtggcacatcttcattcccaattcagaaagtacacattgccctgcacgtctcccacggcaagctgcagggtggagttagcgcccagccaaggttccaggcagctcactgacccttcgcatcggaacaggcccagcagctgcatactgggtctctcccatagcttaacatctctgtccttcgaagctgtcaccagcaactcaggtagcacatggagggctgtgacagagcccgagtgaatctttctacgctgccgtgtctttagatgtggtgttggctcactatccatgctggcatcactatccatgctggcatcagattccctgcaggtagatgggtctgtccctggagtttgggtttctggagtgtttgcttttttctgccacatgttacctgtggtccattctccttctgggctgcatttggccaggttccataggatcccatcagagctggcacacaaaaatgaggactcagattcaggtttggcttgagttatcgatattagggtcctactaggattctctaagtttatatcaaagttcagcctctcttcaaactctcctgattccttttgcctcaagaaagaaagaactccaggatccttgggctgcaggacaaatatgccatactccttgtgggtggacaatatcataggattttctgtatagctgctccagatttcagatggagcatcccctggcttcatgcaaagtaacttcaaatctgctttggccaagatgagaaagtgaccatcaggagcccaatccagacttgtcagcacccctaagtcctcctgtagaattcggttcaggtgaagactcaaatttccgggtgccgaacccttccgcagtttcacttgccactcgctgattttctcatcagcactgaggacaaaaaaggtgtgtgccgaggaccagatcagagcaccaatgtggcctggagcctgtgctgtggccacagccttagcttcctgccacaagattagttccccagcttgatttccagatactgccatggaaccatctggtgcccaagccacagcagtgacggctgcagaactccttggtatacatgtgtcatctgcttccttaggaacctgccagagccgtacagaaccatcctcagaggcggtcagcatgaggcctgaggtttctgaaacagcagcagcacggactgggccgctgtgtcccaggagggtgtgggtttggcacaccaagagtggatgccataaccgtgtggccccatctagcccgacggttaccaccagaagctctgacccaggctgtccagctgcacggggctccatggcagctgcacagtggctaatgggtcctgagtgagcagggatgctggtcagctccacgccttgatggtcccacactttcaaggtcccatcccggctcacagacaccacgtgctcctccacagctgccacagcgctcacagcactctgatgacccaggaactgaccaagccgctgtcctgactctgggtcccagagccccacagagccatcactggagcaggatatcagtaggttatctttggtccaggcacagccagtgacccagtcacggtgacaggcagggaaggagtggatcaaaacaggggttttgggtgtcctcacgtcccagcagaggagactccgatcccggcccccggtggccaggctgcctccatcagtgctgaaactacagcagctcacagggccctcatgtccccgcagctcagtgccacagggaaagtcttctgccttgtgtggccgcgtcagcagctgccttggccacagctgcactgtgaaatcctctgaggcagaagccaagagctcctgggaagtggccagtcctagcacaggcttctggaatctggacaggagccagagggactgaagggagcattccttgagtgcccagccctgcaaggacccatcttctgcaccactcaccaataccttggggcttagccaggccagggcggacactgccacatccagtgcctgaccctgagccccctgggaacctgaagagattttgtagatcctaatgccatccgctcgatatccaacagccacccgatcaccatctgggctgagtgccacagagagggcaggagagagagaaagggaacccaggtgcccacggggccgacccagagaccctgaccacacctgaaccttgccatcctctccagccgtcagtaactggcaacccgcatgcaggaaaagcgcagcagcaacaaagccatggtgggcagggaaggcagccagccgtgccccttctcgccaggcccacagctccaccatactgtccagccggcccacagccacaacccccccaggcacattgaaggccaaggtacggatagaggctccgggtgcccccaggtccttggtgactttgagcccatccacctggaagaagctgatgctgccagcccagctgcctgtggctattacctgcccctctgggtggaaggcaacacagttcagggacttggggtaggtgtgctggaaggccagctgcccacggactgtgtcccacagctttaggcatcctcccaagcacacggtggctagcagccggcagtctgggctcaggcagcagccagtgatttggtactggtgagccttagtctgcagcacccgacaaccatgctgcaggtcccagagctccaggagcccgtcgaaggcagtaagaaagagtgtatcatcggagaggaacaaacaagcagagattccatcacagccactcaccacagacttctcctcctgccaagttctcaggtccaacaggtaaactgtcccattggcagtgcccacagctgctctttgcccattggtggagaaggccacagcagtaggggatgaggaaactgccagagacaggctggagctttgctgatttttcatggtccggggtttattaagccatcgtagtgtgtgttggaggtgccatctccgggagagcagcgaggcttggtggcaaagaggtgagtccaggggctggttggctgcctgctggggcaggagccgggggtactggctgaggattgaagcctgctgcctcaggaaggtgcgaaacactgcaacgtcagcctcggggagcttttgttcctctttggggactgaagaagcatagagggcatgggcctccaagagccgagagaccagacccaattccaagtgtgcagccaccacatggaggttggtaaggaacttcgaaagaagtccacggttcccgctctggagcaggtggtaaggcaggtctcccagagcctcaggagggcaacttcggaaggtgcctgaggcatcagcgtcacatgtcttccagagctgagctgcaatgaggatgtgtgccgtgtcctctagccctggcctcttcccatagcaacgtttagctgctgttctcaggggcccatcagggaggcacagccgggcaccagggcgctccagagggccctcccctagcaaactgcgcagactctggacgaggcaggcaaacgggcccatggggtaggggtctccactgttaccagcagccactgcttcttcccagctcttagtccccttcggtagtgtccgccacacactcagcactccgtgcagctggtccacagtcaaaccactccgtgtgacttctagggcagtcaaggcctggggaaggacatcaggcccgtgctccttctccagtgtgctcaggatgtgctgcagcagcagggggacagtggcaggcagggtccggagtctctcagacacctgctcatacagcgtgaagagcctcaggtgatcggtgaccaagcgcaggtagagcggccggcctgattcccgcttcaccagcagcagtcgcatctggttgttaaatggtgactcctccagccgcttcccgtacagggccagctcctctctcaccagccgggcccgagcagaggcctccagaggccccaaggccagcacgtgggcaccctggctctgctcaagggtctcccctaggcctgcatcactagacacactcagcaccaggtgtacacaccggggaagcttctttgggatccagtctgaaatcagctgcccattctggtccactaacctatcagccccatcgatgatcaggacctgggtctggccaggatgcagggactcagcagacttgggcagcagcctctgctgcagctcccacaccaggcttcggtaggtgctggggagggcacctggctcttttagttggccacgcagataggtacagaggcgtctgagcagagtgagggcaagaccctggtcaggacgagccccagaaaagtggaagaagactaatgatgccaccttggccccatcaggagcctgcagggctgacacaagagatgccaggaaggctgtcttgccctgtcctgactgccccgtcaccaggctcagccttccgtggggcagcatcagccgttgcactgtgtcctgaagaaggcgtggccgggcaggactcggtggcttctgcagctgctggaaggtggcctggaccaagtcatcgtctgggatggacactggctgctccagcagggccccaggctgcaggtagagcttctggatcatattccatacatcctgcagaaccaactgcccaaactcctccagcccgccaacatagggccggccagctgccacacccccccactcacaggggtatctgcggcaggtgatccctttctgtctgcttaggtagctcttcagttctgagatccgacgtgcggcctcttcagactcagaaacaaagtcagatttccaggcatctggcacagagctgaggaagctggaatcccggaagtagatgagagcttgggcagagggctgcagacgttggttccggttcaggaactgcatcacctccatctctgtcacagagcgccctgaagggtactgctgggcccagtggaagtgtggatggtcaggaaggttgtagctggggggaatgtatccataacgggagcccagaatccccacaaacagctgtgcgttctccacctccccaaggcacacttccagttgtctgttcctacgggtctcctcctcagtgacgccccagcggaggtcgattccgtgaaggctgatacggtgaggggccgctcgggcctgcagtgctggcagcacagacctcagcagcaggtcccgctccccatgcatgtctcggaaagtggatgaaatgaaaagccggatgctgcgccatccttgctgggaaacaggagccaaggggcttggagtgtcctcttccagtggccggagagactggacccctgtctttcctgggggtggtggaatcttgaatattttgtccatttggcccacatgttccagaagatgggaggccccatgctctgcaatgaacttcagtatcgcatcagtacagcctgagagtgtcacatcattgggattcaaatctgttgacaggtattgtacccttcttaggaggataccaacaaagaggcacttggaattcacacgctgccagtaaagctgtttggccacatttatcattccatcatccatgctttggccaaggaggatgaccctgtccacaggaaccctttggccagccagagacagcaggtatttcccaaaagtattcagggaccatccatcattttcatcaaactcctggacttgagcctggagcttgatggcagtcttcaggatgccttcttctgccttaagcactgcagtcttcagagtgtcacctccacacagcacgacgtccacctgctccgccctcgtgatcatcatcccaatcaacagcagtgcatagttcagcgggggcccttgtgggttgctctttggacagagcctgtctgcattagcatctgtcagatagaccaagacagtgcggcctggcagcaggggcaggctgtgcttcacagagaggttcacagctgtctctagggcctgtcggtacctgttcagcatctcaccatcatatttccactgtctggccttgtgtactctcagcttctccctcttgagctgctcatacaacacaggtatcctcattgccatccgaagctgctgacggcttaggtggcaaagaaacctccgcctgggacggttcttttcatttctagttagtatccgcctcatcagtgttatattcgaaggaaagggcaatgcttgatttctgagttgagcctcgagggcatcaatggcatcatgggcgttaagaaatctgaatggaaactgccgactgtggatcaccgacttcgcatgctggagtctctggagaatgagctcatggtggcgggaactgattccaacccgcagcaggttgcacaggttccgaagcatggccatgaagggaagcttcccattttctgtaacccagcagggcttgaacgtgctgggcaggcttgtggatgtgcagtcgctgaaccagcttcttcagggt

SEQ ID NO: 11396 - RNA, 8615 nt, Homo sapiens
  source 1..8615: mol_type = other RNA
ctgaatagctgggactacaggtgcccgccgccacacctggctaactttttgtattttttagtagagacagggtttcactatgttagccaggatggtcttgatctcctgacctcgtgatctgcccacctcggcctcccaaagtgctgggattacaagcgtgagccaccatgcccggcctcctctgggtagttctgagaaaagggctgtctctgtgacagaaacatagctctttctaaatgccctgatgcatgactgacttattctccctccctcattctttcccgatgaactgaaaggtcttccatgctctgttcaaattgaatgttggccaacatcactctcattcctcctcctggcaagaatggcatcctagggtcctagggcccgcgagtgatgcaagaattctaaaacctagtttcaaaagagtacctactaaagatttcattcactttcttgtggttctagtaaggattaatgttgaataagaagagacacacattagaatgtacatatacatacacatagaatatcctcctgttctaaatccacatgagaacacaggcaggcctacacttgagattttttgacacttcatttttataattatcaagaaattattaattttataattattaaaagctaccagtgtcttcaggctttgcatctctagcacaaggggtatcattattcccgagtggcacatcttcattcccaattcagaaagtacacattgccctgcacgtctcccacggcaagctgcagggtggagttagcgcccagccaaggttccaggcagctcactgacccttcgcatcggaacaggcccagcagctgcatactgggtctctcccatagcttaacatctctgtccttcgaagctgtcaccagcaactcaggtagcacatggagggctgtgacagagcccgagtgaatctttctacgctgccgtgtctttagatgtggtgttggctcactatccatgctggcatcactatccatgctggcatcagattccctgcaggtagatgggtctgtccctggagtttgggtttctggagtgtttgcttttttctgccacatgttacctgtggtccattctccttctgggctgcatttggccaggttccataggatcccatcagagctggcacacaaaaatgaggactcagattcaggtttggcttgagttatcgatattagggtcctactaggattctctaagtttatatcaaagttcagcctctcttcaaactctcctgattccttttgcctcaagaaagaaagaactccaggatccttgggctgcaggacaaatatgccatactccttgtgggtggacaatatcataggattttctgtatagctgctccagatttcagatggagcatcccctggcttcatgcaaagtaacttcaaatctgctttggccaagatgagaaagtgaccatcaggagcccaatccagacttgtcagcacccctaagtcctcctgtagaattcggttcaggtgaagactcaaatttccgggtgccgaacccttccgcagtttcacttgccactcgctgattttctcatcagcactgaggacaaaaaaggtgtgtgccgaggaccagatcagagcaccaatgtggcctggagcctgtgctgtggccacagccttagcttcctgccacaagattagttccccagcttgatttccagatactgccatggaaccatctggtgcccaagccacagcagtgacggctgcagaactccttggtatacatgtgtcatctgcttccttaggaacctgccagagccgtacagaaccatcctcagaggcggtcagcatgaggcctgaggtttctgaaacagcagcagcacggactgggccgctgtgtcccaggagggtgtgggtttggcacaccaagagtggatgccataaccgtgtggccccatctagcccgacggttaccaccagaagctctgacccaggctgtccagctgcacggggctccatggcagctgcacagtggctaatgggtcctgagtgagcagggatgctggtcagctccacgccttgatggtcccacactttcaaggtcccatcccggctcacagacaccacgtgctcctccacagctgccacagcgctcacagcactctgatgacccaggaactgaccaagccgctgtcctgactctgggtcccagagccccacagagccatcactggagcaggatatcagtaggttatctttggtccaggcacagccagtgacccagtcacggtgacaggcagggaaggagtggatcaaaacaggggttttgggtgtcctcacgtcccagcagaggagactccgatcccggcccccggtggccaggctgcctccatcagtgctgaaactacagcagctcacagggccctcatgtccccgcagctcagtgccacagggaaagtcttctgccttgtgtggccgcgtcagcagctgccttggccacagctgcactgtgaaatcctctgaggcagaagccaagagctcctgggaagtggccagtcctagcacaggcttctggaatctggacaggagccagagggactgaagggagcattccttgagtgcccagccctgcaaggacccatcttctgcaccactcaccaataccttggggcttagccaggccagggcggacactgccacatccagtgcctgaccctgagccccctgggaacctgaagagattttgtagatcctaatgccatccgctcgatatccaacagccacccgatcaccatctgggctgagtgccacagagagggcaggagagagagaaagggaacccaggtgcccacggggccgacccagagaccctgaccacacctgaaccttgccatcctctccagccgtcagtaactggcaacccgcatgcaggaaaagcgcagcagcaacaaagccatggtgggcagggaaggcagccagccgtgccccttctcgccaggcccacagctccaccatactgtccagccggcccacagccacaacccccccaggcacattgaaggccaaggtacggatagaggctccgggtgcccccaggtccttggtgactttgagcccatccacctggaagaagctgatgctgccagcccagctgcctgtggctattacctgcccctctgggtggaaggcaacacagttcagggacttggggtaggtgtgctggaaggccagctgcccacggactgtgtcccacagctttaggcatcctcccaagcacacggtggctagcagccggcagtctgggctcaggcagcagccagtgatttggtactggtgagccttagtctgcagcacccgacaaccatgctgcaggtcccagagctccaggagcccgtcgaaggcagtaagaaagagtgtatcatcggagaggaacaaacaagcagagattccatcacagccactcaccacagacttctcctcctgccaagttctcaggtccaacaggtaaactgtcccattggcagtgcccacagctgctctttgcccattggtggagaaggccacagcagtaggggatgaggaaactgccagagacaggctggagctttgctgatttttcatggtccggggtttattaagccatcgtagtgtgtgttggaggtgccatctccgggagagcagcgaggcttggtggcaaagaggtgagtccaggggctggttggctgcctgctggggcaggagccgggggtactggctgaggattgaagcctgctgcctcaggaaggtgcgaaacactgcaacgtcagcctcggggagcttttgttcctctttggggactgaagaagcatagagggcatgggcctccaagagccgagagaccagacccaattccaagtgtgcagccaccacatggaggttggtaaggaacttcgaaagaagtccacggttcccgctctggagcaggtggtaaggcaggtctcccagagcctcaggagggcaacttcggaaggtgcctgaggcatcagcgtcacatgtcttccagagctgagctgcgcagactctggacgaggcaggcaaacgggcccatggggtaggggtctccactgttaccagcagccactgcttcttcccagctcttagtccccttcggtagtgtccgccacacactcagcactccgtgcagctggtccacagtcaaaccactccgtgtgacttctagggcagtcaaggcctggggaaggacatcaggcccgtgctccttctccagtgtgctcaggatgtgctgcagcagcagggggacagtggcaggcagggtccggagtctctcagacacctgctcatacagcgtgaagagcctcaggtgatcggtgaccaagcgcaggtagagcggccggcctgattcccgcttcaccagcagcagtcgcatctggttgttaaatggtgactcctccagccgcttcccgtacagggccagctcctctctcaccagccgggcccgagcagaggcctccagaggccccaaggccagcacgtgggcaccctggctctgctcaagggtctcccctaggcctgcatcactagacacactcagcaccaggtgtacacaccggggaagcttctttgggatccagtctgaaatcagctgcccattctggtccactaacctatcagccccatcgatgatcaggacctgggtctggccaggatgcagggactcagcagacttgggcagcagcctctgctgcagctcccacaccaggcttcggtaggtgctggggagggcacctggctcttttagttggccacgcagataggtacagaggcgtctgagcagagtgagggcaagaccctggtcaggacgagccccagaaaagtggaagaagactaatgatgccaccttggccccatcaggagcctgcagggctgacacaagagatgccaggaaggctgtcttgccctgtcctgactgccccgtcaccaggctcagccttccgtggggcagcatcagccgttgcactgtgtcctgaagaaggcgtggccgggcaggactcggtggcttctgcagctgctggaaggtggcctggaccaagtcatcgtctgggatggacactggctgctccagcagggccccaggctgcaggtagagcttctggatcatattccatacatcctgcagaaccaactgcccaaactcctccagcccgccaacatagggccggccagctgccacacccccccactcacaggggtatctgcggcaggtgatccctttctgtctgcttaggtagctcttcagttctgagatccgacgtgcggcctcttcagactcagaaacaaagtcagatttccaggcatctggcacagagctgaggaagctggaatcccggaagtagatgagagcttgggcagagggctgcagacgttggttccggttcaggaactgcatcacctccatctctgtcacagagcgccctgaagggtactgctgggcccagtggaagtgtggatggtcaggaaggttgtagctggggggaatgtatccataacgggagcccagaatccccacaaacagctgtgcgttctccacctccccaaggcacacttccagttgtctgttcctacgggtctcctcctcagtgacgccccagcggaggtcgattccgtgaaggctgatacggtgaggggccgctcgggcctgcagtgctggcagcacagacctcagcagcaggtcccgctccccatgcatgtctcggaaagtggatgaaatgaaaagccggatgctgcgccatccttgctgggaaacaggagccaaggggcttggagtgtcctcttccagtggccggagagactggacccctgtctttcctgggggtggtggaatcttgaatattttgtccatttggcccacatgttccagaagatgggaggccccatgctctgcaatgaacttcagtatcgcatcagtacagcctgagagtgtcacatcattgggattcaaatctgttgacaggtattgtacccttcttaggaggataccaacaaagaggcacttggaattcacacgctgccagtaaagctgtttggccacatttatcattccatcatccatgctttggccaaggaggatgaccctgtccacaggaaccctttggccagccagagacagcaggtatttcccaaaagtattcagggaccatccatcattttcatcaaactcctggacttgagcctggagcttgatggcagtcttcaggatgccttcttctgccttaagcactgcagtcttcagagtgtcacctccacacagcacgacgtccacctgctccgccctcgtgatcatcatcccaatcaacagcagtgcatagttcagcgggggcccttgtgggttgctctttggacagagcctgtctgcattagcatctgtcagatagaccaagacagtgcggcctggcagcaggggcaggctgtgcttcacagagaggttcacagctgtctctagggcctgtcggtacctgttcagcatctcaccatcatatttccactgtctggccttgtgtactctcagcttctccctcttgagctgctcatacaacacaggtatcctcattgccatccgaagctgctgacggcttaggtggcaaagaaacctccgcctgggacggttcttttcatttctagttagtatccgcctcatcagtgttatattcgaaggaaagggcaatgcttgatttctgagttgagcctcgagggcatcaatggcatcatgggcgttaagaaatctgaatggaaactgccgactgtggatcaccgacttcgcatgctggagtctctggagaatgagctcatggtggcgggaactgattccaacccgcagcaggttgcacaggttccgaagcatggccatgaagggaagcttcccattttcaatgagttcctcccagaccgacgctttgttcccccgtaggctcagctcccgctcccaggtctctggcctagacagcttcatcctcttcccagctctgctagaatcccaaggcccaggaaggcgacttcgagaaaagagctgtaggttggaggggtatctgtaacccagcagggcttgaacgtgctgggcaggcttgtggatgtgcagtcgctgaaccagcttcttcagggtgaaccttggaggattctttttctctgacactgtatcaccggccttctcaaactttctctgctcttctctgagaaaccctatgtaccttggaaaacatctgtgagaaaatggaggctccatccctggagagcggggtggccggcgggggtgtctcttggcccggtgcttccgagggttgtacttagccagctggtactcgtcaaactgggcaaatttgtccgtcatggcagtacggagacaggcgggcaggggcaccagcttattcttatctccctcagccaggctctggtaaagctcagccacctggatccagtcagaaggcagctggacaatggcacagaaatatcgtcgcaggtgggggcgacacgccggcaagaaagcagcaatggccaagatgttattggccacattccggacgttcagctgctgcctggcatacaaagatgccttgaggataaactcaggctccaggagggcaagttcacgacagatttcaaaaatggcagccagggtggggtcagatgtattgttcatgtttacttctgagaccagagtagagcacagcaagctcagtagagccatcttcttttcctgaaggacatggtcagtaggctctggatgagattcagagtctccagaggtgagcttcacggccagatcctccacctcctcctcctctcccaagctcagactataagaaggcatttgggtctctgcccctttcttctcttctgaatcaaaccaacgacccaaagttgcttcctgagctgtctctgtggcagagatggatttcagggctatagggcaggttgaaaggtctagtcccttagagaaatgctgagccctccaacttggaggctcagagagcaggcaattgctgttgttcacacggtacaaatcagcttgcgtcatgtgagatatctgtagactctggaacaaggggctggcagacacagtgctctttagactagagagggtggccaggcaccggttctccaaggagaggatgtctgggtgggcagaaacatgtccatgtggtttctccatggtcttcaggtcagaaagtgtggccaggcactggttctccaaggagaggatgtctgggtgggcagacacatatccatgtggtttttccatggtcttcaggtcaggaagcgtggctaggcactggttcttcaaggagaggatatctgagtgggtagatacatgctgatgtagtttctccaagggctgtaagtcagggagcatagccaggcaccggttctccaaggagaggatgtctggatgggcagacacatgcccatggagtttttccatggctgaaactcagcttgtatatgcctggggcgtccgattcccgcagcaggaagcagaaacttcgctctggattctgccggtgggaagggtggcagccgggggaggagccggatgcggatctgagaagagacggtgcgggcggagactctcgggcccgggc

SEQ ID NO: 11397 - RNA, 8652 nt, Homo sapiens
  source 1..8652: mol_type = other RNA
ctgaatagctgggactacaggtgcccgccgccacacctggctaactttttgtattttttagtagagacagggtttcactatgttagccaggatggtcttgatctcctgacctcgtgatctgcccacctcggcctcccaaagtgctgggattacaagcgtgagccaccatgcccggcctcctctgggtagttctgagaaaagggctgtctctgtgacagaaacatagctctttctaaatgccctgatgcatgactgacttattctccctccctcattctttcccgatgaactgaaaggtcttccatgctctgttcaaattgaatgttggccaacatcactctcattcctcctcctggcaagaatggcatcctagggtcctagggcccgcgagtgatgcaagaattctaaaacctagtttcaaaagagtacctactaaagatttcattcactttcttgtggttctagtaaggattaatgttgaataagaagagacacacattagaatgtacatatacatacacatagaatatcctcctgttctaaatccacatgagaacacaggcaggcctacacttgagattttttgacacttcatttttataattatcaagaaattattaattttataattattaaaagctaccagtgtcttcaggctttgcatctctagcacaaggggtatcattattcccgagtggcacatcttcattcccaattcagaaagtacacattgccctgcacgtctcccacggcaagctgcagggtggagttagcgcccagccaaggttccaggcagctcactgacccttcgcatcggaacaggcccagcagctgcatactgggtctctcccatagcttaacatctctgtccttcgaagctgtcaccagcaactcaggtagcacatggagggctgtgacagagcccgagtgaatctttctacgctgccgtgtctttagatgtggtgttggctcactatccatgctggcatcactatccatgctggcatcagattccctgcaggtagatgggtctgtccctggagtttgggtttctggagtgtttgcttttttctgccacatgttacctgtggtccattctccttctgggctgcatttggccaggttccataggatcccatcagagctggcacacaaaaatgaggactcagattcaggtttggcttgagttatcgatattagggtcctactaggattctctaagtttatatcaaagttcagcctctcttcaaactctcctgattccttttgcctcaagaaagaaagaactccaggatccttgggctgcaggacaaatatgccatactccttgtgggtggacaatatcataggattttctgtatagctgctccagatttcagatggagcatcccctggcttcatgcaaagtaacttcaaatctgctttggccaagatgagaaagtgaccatcaggagcccaatccagacttgtcagcacccctaagtcctcctgtagaattcggttcaggtgaagactgtgctgtggccacagccttagcttcctgccacaagattagttccccagcttgatttccagatactgccatggaaccatctggtgcccaagccacagcagtgacggctgcagaactccttggtatacatgtgtcatctgcttccttaggaacctgccagagccgtacagaaccatcctcagaggcggtcagcatgaggcctgaggtttctgaaacagcagcagcacggactgggccgctgtgtcccaggagggtgtgggtttggcacaccaagagtggatgccataaccgtgtggccccatctagcccgacggttaccaccagaagctctgacccaggctgtccagctgcacggggctccatggcagctgcacagtggctaatgggtcctgagtgagcagggatgctggtcagctccacgccttgatggtcccacactttcaaggtcccatcccggctcacagacaccacgtgctcctccacagctgccacagcgctcacagcactctgatgacccaggaactgaccaagccgctgtcctgactctgggtcccagagccccacagagccatcactggagcaggatatcagtaggttatctttggtccaggcacagccagtgacccagtcacggtgacaggcagggaaggagtggatcaaaacaggggttttgggtgtcctcacgtcccagcagaggagactccgatcccggcccccggtggccaggctgcctccatcagtgctgaaactacagcagctcacagggccctcatgtccccgcagctcagtgccacagggaaagtcttctgccttgtgtggccgcgtcagcagctgccttggccacagctgcactgtgaaatcctctgaggcagaagccaagagctcctgggaagtggccagtcctagcacaggcttctggaatctggacaggagccagagggactgaagggagcattccttgagtgcccagccctgcaaggacccatcttctgcaccactcaccaataccttggggcttagccaggccagggcggacactgccacatccagtgcctgaccctgagccccctgggaacctgaagagattttgtagatcctaatgccatccgctcgatatccaacagccacccgatcaccatctgggctgagtgccacagagagggcaggagagagagaaagggaacccaggtgcccacggggccgacccagagaccctgaccacacctgaaccttgccatcctctccagccgtcagtaactggcaacccgcatgcaggaaaagcgcagcagcaacaaagccatggtgggcagggaaggcagccagccgtgccccttctcgccaggcccacagctccaccatactgtccagccggcccacagccacaacccccccaggcacattgaaggccaaggtacggatagaggctccgggtgcccccaggtccttggtgactttgagcccatccacctggaagaagctgatgctgccagcccagctgcctgtggctattacctgcccctctgggtggaaggcaacacagttcagggacttggggtaggtgtgctggaaggccagctgcccacggactgtgtcccacagctttaggcatcctcccaagcacacggtggctagcagccggcagtctgggctcaggcagcagccagtgatttggtactggtgagccttagtctgcagcacccgacaaccatgctgcaggtcccagagctccaggagcccgtcgaaggcagtaagaaagagtgtatcatcggagaggaacaaacaagcagagattccatcacagccactcaccacagacttctcctcctgccaagttctcaggtccaacaggtaaactgtcccattggcagtgcccacagctgctctttgcccattggtggagaaggccacagcagtaggggatgaggaaactgccagagacaggctggagctttgctgatttttcatggtccggggtttattaagccatcgtagtgtgtgttggaggtgccatctccgggagagcagcgaggcttggtggcaaagaggtgagtccaggggctggttggctgcctgctggggcaggagccgggggtactggctgaggattgaagcctgctgcctcaggaaggtgcgaaacactgcaacgtcagcctcggggagcttttgttcctctttggggactgaagaagcatagagggcatgggcctccaagagccgagagaccagacccaattccaagtgtgcagccaccacatggaggttggtaaggaacttcgaaagaagtccacggttcccgctctggagcaggtggtaaggcaggtctcccagagcctcaggagggcaacttcggaaggtgcctgaggcatcagcgtcacatgtcttccagagctgagctgcaatgaggatgtgtgccgtgtcctctagccctggcctcttcccatagcaacgtttagctgctgttctcaggggcccatcagggaggcacagccgggcaccagggcgctccagagggccctcccctagcaaactgcgcagactctggacgaggcaggcaaacgggcccatggggtaggggtctccactgttaccagcagccactgcttcttcccagctcttagtccccttcggtagtgtccgccacacactcagcactccgtgcagctggtccacagtcaaaccactccgtgtgacttctagggcagtcaaggcctggggaaggacatcaggcccgtgctccttctccagtgtgctcaggatgtgctgcagcagcagggggacagtggcaggcagggtccggagtctctcagacacctgctcatacagcgtgaagagcctcaggtgatcggtgaccaagcgcaggtagagcggccggcctgattcccgcttcaccagcagcagtcgcatctggttgttaaatggtgactcctccagccgcttcccgtacagggccagctcctctctcaccagccgggcccgagcagaggcctccagaggccccaaggccagcacgtgggcaccctggctctgctcaagggtctcccctaggcctgcatcactagacacactcagcaccaggtgtacacaccggggaagcttctttgggatccagtctgaaatcagctgcccattctggtccactaacctatcagccccatcgatgatcaggacctgggtctggccaggatgcagggactcagcagacttgggcagcagcctctgctgcagctcccacaccaggcttcggtaggtgctggggagggcacctggctcttttagttggccacgcagataggtacagaggcgtctgagcagagtgagggcaagaccctggtcaggacgagccccagaaaagtggaagaagactaatgatgccaccttggccccatcaggagcctgcagggctgacacaagagatgccaggaaggctgtcttgccctgtcctgactgccccgtcaccaggctcagccttccgtggggcagcatcagccgttgcactgtgtcctgaagaaggcgtggccgggcaggactcggtggcttctgcagctgctggaaggtggcctggaccaagtcatcgtctgggatggacactggctgctccagcagggccccaggctgcaggtagagcttctggatcatattccatacatcctgcagaaccaactgcccaaactcctccagcccgccaacatagggccggccagctgccacacccccccactcacaggggtatctgcggcaggtgatccctttctgtctgcttaggtagctcttcagttctgagatccgacgtgcggcctcttcagactcagaaacaaagtcagatttccaggcatctggcacagagctgaggaagctggaatcccggaagtagatgagagcttgggcagagggctgcagacgttggttccggttcaggaactgcatcacctccatctctgtcacagagcgccctgaagggtactgctgggcccagtggaagtgtggatggtcaggaaggttgtagctggggggaatgtatccataacgggagcccagaatccccacaaacagctgtgcgttctccacctccccaaggcacacttccagttgtctgttcctacgggtctcctcctcagtgacgccccagcggaggtcgattccgtgaaggctgatacggtgaggggccgctcgggcctgcagtgctggcagcacagacctcagcagcaggtcccgctccccatgcatgtctcggaaagtggatgaaatgaaaagccggatgctgcgccatccttgctgggaaacaggagccaaggggcttggagtgtcctcttccagtggccggagagactggacccctgtctttcctgggggtggtggaatcttgaatattttgtccatttggcccacatgttccagaagatgggaggccccatgctctgcaatgaacttcagtatcgcatcagtacagcctgagagtgtcacatcattgggattcaaatctgttgacaggtattgtacccttcttaggaggataccaacaaagaggcacttggaattcacacgctgccagtaaagctgtttggccacatttatcattccatcatccatgctttggccaaggaggatgaccctgtccacaggaaccctttggccagccagagacagcaggtatttcccaaaagtattcagggaccatccatcattttcatcaaactcctggacttgagcctggagcttgatggcagtcttcaggatgccttcttctgccttaagcactgcagtcttcagagtgtcacctccacacagcacgacgtccacctgctccgccctcgtgatcatcatcccaatcaacagcagtgcatagttcagcgggggcccttgtgggttgctctttggacagagcctgtctgcattagcatctgtcagatagaccaagacagtgcggcctggcagcaggggcaggctgtgcttcacagagaggttcacagctgtctctagggcctgtcggtacctgttcagcatctcaccatcatatttccactgtctggccttgtgtactctcagcttctccctcttgagctgctcatacaacacaggtatcctcattgccatccgaagctgctgacggcttaggtggcaaagaaacctccgcctgggacggttcttttcatttctagttagtatccgcctcatcagtgttatattcgaaggaaagggcaatgcttgatttctgagttgagcctcgagggcatcaatggcatcatgggcgttaagaaatctgaatggaaactgccgactgtggatcaccgacttcgcatgctggagtctctggagaatgagctcatggtggcgggaactgattccaacccgcagcaggttgcacaggttccgaagcatggccatgaagggaagcttcccattttcaatgagttcctcccagaccgacgctttgttcccccgtaggctcagctcccgctcccaggtctctggcctagacagcttcatcctcttcccagctctgctagaatcccaaggcccaggaaggcgacttcgagaaaagagctgtaggttggaggggtatctgtaacccagcagggcttgaacgtgctgggcaggcttgtggatgtgcagtcgctgaaccagcttcttcagggtgaaccttggaggattctttttctctgacactgtatcaccggccttctcaaactttctctgctcttctctgagaaaccctatgtaccttggaaaacatctgtgagaaaatggaggctccatccctggagagcggggtggccggcgggggtgtctcttggcccggtgcttccgagggttgtacttagccagctggtactcgtcaaactgggcaaatttgtccgtcatggcagtacggagacaggcgggcaggggcaccagcttattcttatctccctcagccaggctctggtaaagctcagccacctggatccagtcagaaggcagctggacaatggcacagaaatatcgtcgcaggtgggggcgacacgccggcaagaaagcagcaatggccaagatgttattggccacattccggacgttcagctgctgcctggcatacaaagatgccttgaggataaactcaggctccaggagggcaagttcacgacagatttcaaaaatggcagccagggtggggtcagatgtattgttcatgtttacttctgagaccagagtagagcacagcaagctcagtagagccatcttcttttcctgaaggacatggtcagtaggctctggatgagattcagagtctccagaggtgagcttcacggccagatcctccacctcctcctcctctcccaagctcagactataagaaggcatttgggtctctgcccctttcttctcttctgaatcaaaccaacgacccaaagttgcttcctgagctgtctctgtggcagagatggatttcagggctatagggcaggttgaaaggtctagtcccttagagaaatgctgagccctccaacttggaggctcagagagcaggcaattgctgttgttcacacggtacaaatcagcttgcgtcatgtgagatatctgtagactctggaacaaggggctggcagacacagtgctctttagactagagagggtggccaggcaccggttctccaaggagaggatgtctgggtgggcagaaacatgtccatgtggtttctccatggtcttcaggtcagaaagtgtggccaggcactggttctccaaggagaggatgtctgggtgggcagacacatatccatgtggtttttccatggtcttcaggtcaggaagcgtggctaggcactggttcttcaaggagaggatatctgagtgggtagatacatgctgatgtagtttctccaagggctgtaagtcagggagcatagccaggcaccggttctccaaggagaggatgtctggatgggcagacacatgcccatggagtttttccatggctgaaactcagcttgtatatgccttagactggggctggaaaccctgggtgcctgacctggggcgtccgattcccgcagcaggaagcagaaacttcgctctggattctgccggtgggaagggtggcagccgggggaggagccggatgcggatctgagaagagacggtgcgggcggagactctcgggc

SEQ ID NO: 11398 - RNA, 2179 nt, Homo sapiens
  source 1..2179: mol_type = other RNA
ctgaatagctgggactacaggtgcccgctctcacgccaggccaatttttgtatttttactaagacggggttgcaccatgttggccaggctggtcttgaactcctgaccttaggtgatccacccgcctcccaaagtgctgggatcacaggcatgagccaccgcacccagccagaagacagctgcttaaaaaagtaattctaaaagctctgacgtcggatcccctctgctgcgttttttgttagtatcaaactgtctttcagagggttaagggagaaaacaaaacccatgatgctccttcacttgctctccgaggcgcaggcgcacagaaacagcggccacggaccacagaaatgcaggacggagctctcctgctcccacgccacgaggctggaacatcagccccagtgcctggtgcacacacaggctcaggaaaactagctccttccatcaagttaaaaacatctcaatccataatcactctgcttataaatactatttgcacttaattggaaaatgtaaaaatcctaggtcttactactagataaacactcatttcataagtactagtttcagaatatgaaatctaatatatttagcatactatgaattgacaataaactgatatgaaatatttaagttcacagtacacatataaagcttcatattatcgcatattaaaaaaaaacagaaagcagcttagagcaatttataacctctaactaaattcctcggtttacaaagtgctttgaaagaccccagctcccagtggcctagtcacagtagtgtcaggaccacaaactgctgtgatcacagcgccgcgtggatcccggaggcaccaggcccctcagggacaggcaggcgggttctgtgggtttgcatttaaggtttttgaggaaaataccttgaaaccgtcggtaggactagataggtgacaacgtgtgacaggaaaggctgtcaggccaagcgcaggcggggctcccagcctcatgataacgtgtaacaggaagggctcccagcctcggtcctcacgtcggtggcaccagaagcgagtgacgacatgtccgtggtcaggaggagcgctggagccagggtgcccagcaggaggtggctgtccccgctgaggtcaccactgcaggggctggcccttgcagtaggggcactcaggtgcggtggccgcacacggctcacagaggatgtggtgctgacagggccgcaggacagcaccgtgggcccgctcccggcaggccacacactgcttggcgcggagctggaagatcaccgtccaccgcctccaggtccaggcgcagctgactctgcagcgagtgcagcttcggcaggggaatggtgccgatgtccccacagccccgcagccccggcagtgtggaggctacgcccaggccctccagctcctcctgcagctgcttcacctgtgcctccacctcctccttcttctgcagcgccagctgccggtcgctatcggccacacgggcacgctccttggcctcctgcgcctctcgctgccaggcatcgcagacctgcttcacctgctgccaggactcctcccactgccggatcttcctcttggcctcgtccagctgccgcctgacccgggccagctcagctccgtttggacttgcactcgaagaggatggggggccggcactcaggatgggggaggggctgggggagaagctgccggaaacaaagtcccagatgctcccggggacaccgttcaaacctagggggctgtaggatgaggctgcagagcccagtgtgcccggctctgaacgcaggggtggcggctgctggggaggcgtcatggctgaggagcccaccggccctgggaggggctgggacagcgaaccgagcggcgaggtggacgcagaggatggcgagtgtagcgatggtgctctgggcagggagccggggatggcgacaggtgcagagccggccagcgacctgggacctgctgctcccaggtcgtggccgtcttgctcttccaggtccttctctagggatgcaatattcacattgctaagatgcaggtctaacgcagaacctggcggggggcgcacctaagggagggcccgctcctgaccgccgagtaacgagacccgcaccttggcggcgcacggctgccacgcgctggggccgccgccaatgctgactcacggtccgc

SEQ ID NO: 11399 - RNA, 3293 nt, Homo sapiens
  source 1..3293: mol_type = other RNA
ctgaatagctgggactacaggtgcccgctctcacgccaggccaatttttgtatttttactaagacggggttgcaccatgttggccaggctggtcttgaactcctgaccttaggtgatccacccgcctcccaaagtgctgggatcacaggcatgagccaccgcacccagccagaagacagctgcttaaaaaagtaattctaaaagctctgacgtcggatcccctctgctgcgttttttgttagtatcaaactgtctttcagagggttaagggagaaaacaaaacccatgatgctccttcacttgctctccgaggcgcaggcgcacagaaacagcggccacggaccacagaaatgcaggacggagctctcctgctcccacgccacgaggctggaacatcagccccagtgcctggtgcacacacaggctcaggaaaactagctccttccatcaagttaaaaacatctcaatccataatcactctgcttataaatactatttgcacttaattggaaaatgtaaaaatcctaggtcttactactagataaacactcatttcataagtactagtttcagaatatgaaatctaatatatttagcatactatgaattgacaataaactgatatgaaatatttaagttcacagtacacatataaagcttcatattatcgcatattaaaaaaaaacagaaagcagcttagagcaatttataacctctaactaaattcctcggtttacaaagtgctttgaaagaccccagctcccagtggcctagtcacagtagtgtcaggaccacaaactgctgtgatcacagcgccgcgtggatcccggaggcaccaggcccctcagggacaggcaggcgggttctgtgggtttgcatttaaggtttttgaggaaaataccttgaaaccgtcggtaggactagataggtgacaacgtgtgacaggaaaggctgtcaggccaagcgcaggcggggctcccagcctcatgataacgtgtaacaggaagggctcccagcctcggtcctcacgtcggtggcaccagaagcgagtgacgacatgtccgtggtcaggaggagcgctggagccagggtgcccagcaggaggtggctgtccccgctgaggtcaccactgcaggggctggcccttgcagtaggggcactcaggtgcggtggccgcacacggctcacagaggatgtggtgctgacagggccgcaggacagcaccgtgggcccgctcccggcaggccacacactgcttggcgcggagctggaagatcacctgtgcctccacctcctccttcttctgcagcgccagctgccggtcgctatcggccacacgggcacgctccttggcctcctgcgcctctcgctgccaggcatcgcagacctgcttcacctgctgccaggactcctcccactgccggatcttcctcttggcctcgtccagctgccgcctgacccgggccagctcagctccgtttggacttgcactcgaagaggatggggggccggcactcaggatgggggaggggctgggggagaagctgccggaaacaaagtcccagatgctcccggggacaccgttcaaacctagggggctgtaggatgaggctgcagagcccagtgtgcccggctctgaacgcaggggtggcggctgctggggaggcgtcatggctgaggagcccaccggccctgggaggggctgggacagcgaaccgagcggcgaggtggacgcagaggatggcgagtgtagcgatggtgctctgggcagggagccggggatggcgacaggtgcagagccggccagcgacctgggacctgctgctcccaggtcgtggccgtcttgctcttccaggtccttctctagggatgcaatattcacattgctaagatgcaggtctaacgcagaaccgaggacggcctccacagtgctgctggcggggccgagcgggagggcacgggcggggggcgcgggcagcgcagtgggggaggagctgccggagccggcgctggacgccaggctggacgccacgctggagctcacgctgggggccggcgggtggaccgctgcaaacacggccaggtggttctgcttgctgtcttgctcgctgcccctagggccaccctcggccggcgagtctctccgcttggcatttcccggctggccgctgcccgtggaggaaggactcgtgaggtggaggtcgtgacagccccattcattcaccatccccaggctcttctcaacgtgtgcaaaggcacagaaggggccgcgcgggcagtacccggtttggcgcatgtcgttgcattttgtagatttgtagatctcgggatggaactgctgctccgtgcgggagtggcaatactggcagccgtcgccgccatcgcagcgtgagggttccccccactcatccccgtgcttcacactggggcagggcgtggacctcctggggacagtgaggccgggcgcccagacagcacggggctgtctcctcgccaactttctgtactggaaccgccgggggttgcgccgcctgtcccggctattgtggtagtgtgggcacgcatagccctggcggcacaggcgtggcggcttcgggcactgctccgtcttgtagctgcccagcacgaagttggcatcttgccaccgggggtcctcgctcaggatcttctcaatcatggcctggctggccaagaccccaggctgcagatccgggaccccttccccgccgcccagctggccgttctgcaaggcttcctgggcctgcagctccctgacgtcacacacgggcggccgcaggtccagggggccgtgcgcgaaggcacagtgcagcccattcttcacgcagtggccacgtgcgtctgtctcgtggatgcaggttcctgttttgtagtaacgcaggtggtacttgcgttctgtgtcccccgtcgtccggtgcaggtagggacactcgtcgccgtcggggcacacgccggtggcttcgttgtacttggagcagtacacgtcggggctgtagttgaaggtgccgtcgcgcctgcggaggggcctgcggcgccgctggttgaggaagtgccagtggaagcaggtgaacggccggtgctgcgcgcacttgtgctgtgaaaacagggggcactgctccgtcctgaactccttcaggtacctgtagtgggtcggcttctcagtctgcgggggggacccgctcagcgccgctgccgccgctttcgaaaccgacggcattttcagtcaaaacaatgcagcgcgcatgcgccgcgccggcgcccccgcccccggatat

SEQ ID NO: 11400 - RNA, 3188 nt, Homo sapiens
  source 1..3188: mol_type = other RNA
ctgaatagctgggactacaggtgcccgctctcacgccaggccaatttttgtatttttactaagacggggttgcaccatgttggccaggctggtcttgaactcctgaccttaggtgatccacccgcctcccaaagtgctgggatcacaggcatgagccaccgcacccagccagaagacagctgcttaaaaaagtaattctaaaagctctgacgtcggatcccctctgctgcgttttttgttagtatcaaactgtctttcagagggttaagggagaaaacaaaacccatgatgctccttcacttgctctccgaggcgcaggcgcacagaaacagcggccacggaccacagaaatgcaggacggagctctcctgctcccacgccacgaggctggaacatcagccccagtgcctggtgcacacacaggctcaggaaaactagctccttccatcaagttaaaaacatctcaatccataatcactctgcttataaatactatttgcacttaattggaaaatgtaaaaatcctaggtcttactactagataaacactcatttcataagtactagtttcagaatatgaaatctaatatatttagcatactatgaattgacaataaactgatatgaaatatttaagttcacagtacacatataaagcttcatattatcgcatattaaaaaaaaacagaaagcagcttagagcaatttataacctctaactaaattcctcggtttacaaagtgctttgaaagaccccagctcccagtggcctagtcacagtagtgtcaggaccacaaactgctgtgatcacagcgccgcgtggatcccggaggcaccaggcccctcagggacaggcaggcgggttctgtgggtttgcatttaaggtttttgaggaaaataccttgaaaccgtcggtaggactagataggtgacaacgtgtgacaggaaaggctgtcaggccaagcgcaggcggggctcccagcctcatgataacgtgtaacaggaagggctcccagcctcggtcctcacgtcggtggcaccagaagcgagtgacgacatgtccgtggtcaggaggagcgctggagccagggtgcccagcaggaggtggctgtccccgctgaggtcaccactgcaggggctggcccttgcagtaggggcactcaggtgcggtggccgcacacggctcacagaggatgtggtgctgacagggccgcaggacagcaccgtgggcccgctcccggcaggccacacactgcttggcgcggagctggaagatcacctgtgcctccacctcctccttcttctgcagcgccagctgccggtcgctatcggccacacgggcacgctccttggcctcctgcgcctctcgctgccaggcatcgcagacctgcttcacctgctgccaggactcctcccactgccggatcttcctcttggcctcgtccagctgccgcctgacccgggccagctcagctccgtttggacttgcactcgaagaggatggggggccggcactcaggatgggggaggggctgggggagaagctgccggaaacaaagtcccagatgctcccggggacaccgttcaaacctagggggctgtaggatgaggctgcagagcccagtgtgcccggctctgaacgcaggggtggcggctgctggggaggcgtcatggctgaggagcccaccggccctgggaggggctgggacagcgaaccgagcggcgaggtggacgcagaggatggcgagtgtagcgatggtgctctgggcagggagccggggatggcgacaggtgcagagccggccagcgacctgggacctgctgctcccaggtcgtggccgtcttgctcttccaggtccttctctagggatgcaatattcacattgctaagatgcaggtctaacgcagaaccgaggacggcctccacagtgctgctggcggggccgagcgggagggcacgggcggggggcgcgggcagcgcagtgggggaggagctgccggagccggcgctggacgccaggctggacgccacgctggagctcacgctgggggccggcgggtggaccgctgcaaacacggccaggtggttctgcttgctgtcttgctcgctgcccctagggccaccctcggccggcgagtctctccgcttggcatttcccggctggccgctgcccgtggaggaaggactcgtgaggtggaggtcgtgacagccccattcattcaccatccccaggctcttctcaacgtgtgcaaaggcacagaaggggccgcgcgggcagtacccggtttggcgcatgtcgttgcattttgtagatttgtagatctcgggatggaactgctgctccgtgcgggagtggcaatactggcagccgtcgccgccatcgcagcgtgagggttccccccactcatccccgtgcttcacactggggcagggcgtggacctgtactggaaccgccgggggttgcgccgcctgtcccggctattgtggtagtgtgggcacgcatagccctggcggcacaggcgtggcggcttcgggcactgctccgtcttgtagctgcccagcacgaagttggcatcttgccaccgggggtcctcgctcaggatcttctcaatcatggcctggctggccaagaccccaggctgcagatccgggaccccttccccgccgcccagctggccgttctgcaaggcttcctgggcctgcagctccctgacgtcacacacgggcggccgcaggtccagggggccgtgcgcgaaggcacagtgcagcccattcttcacgcagtggccacgtgcgtctgtctcgtggatgcaggttcctgttttgtagtaacgcaggtggtacttgcgttctgtgtcccccgtcgtccggtgcaggtagggacactcgtcgccgtcggggcacacgccggtggcttcgttgtacttggagcagtacacgtcggggctgtagttgaaggtgccgtcgcgcctgcggaggggcctgcggcgccgctggttgaggaagtgccagtggaagcaggtgaacggccggtgctgcgcgcacttgtgctgtgaaaacagggggcactgctccgtcctgaactccttcaggtacctgtagtgggtcggcttctcagtctgcgggggggacccgctcagcgccgctgccgccgctttcgaaaccgacggcattttcagtcaaaac

SEQ ID NO: 11401 - RNA, 2031 nt, Homo sapiens
  source 1..2031: mol_type = other RNA
ctgaatagctgggactacaggtgcccgctctcacgccaggccaatttttgtatttttactaagacggggttgcaccatgttggccaggctggtcttgaactcctgaccttaggtgatccacccgcctcccaaagtgctgggatcacaggcatgagccaccgcacccagccagaagacagctgcttaaaaaagtaattctaaaagctctgacgtcggatcccctctgctgcgttttttgttagtatcaaactgtctttcagagggttaagggagaaaacaaaacccatgatgctccttcacttgctctccgaggcgcaggcgcacagaaacagcggccacggaccacagaaatgcaggacggagctctcctgctcccacgccacgaggctggaacatcagccccagtgcctggtgcacacacaggctcaggaaaactagctccttccatcaagttaaaaacatctcaatccataatcactctgcttataaatactatttgcacttaattggaaaatgtaaaaatcctaggtcttactactagataaacactcatttcataagtactagtttcagaatatgaaatctaatatatttagcatactatgaattgacaataaactgatatgaaatatttaagttcacagtacacatataaagcttcatattatcgcatattaaaaaaaaacagaaagcagcttagagcaatttataacctctaactaaattcctcggtttacaaagtgctttgaaagaccccagctcccagtggcctagtcacagtagtgtcaggaccacaaactgctgtgatcacagcgccgcgtggatcccggaggcaccaggcccctcagggacaggcaggcgggttctgtgggtttgcatttaaggtttttgaggaaaataccttgaaaccgtcggtaggactagataggtgacaacgtgtgacaggaaaggctgtcaggccaagcgcaggcggggctcccagcctcatgataacgtgtaacaggaagggctcccagcctcggtcctcacgtcggtggcaccagaagcgagtgacgacatgtccgtggtcaggaggagcgctggagccagggtgcccagcaggaggtggctgtccccgctgaggtcaccactgcaggggctggcccttgcagtaggggcactcaggtgcggtggccgcacacggctcacagaggatgtggtgctgacagggccgcaggacagcaccgtgggcccgctcccggcaggccacacactgcttggcgcggagctggaagatcacctgtgcctccacctcctccttcttctgcagcgccagctgccggtcgctatcggccacacgggcacgctccttggcctcctgcgcctctcgctgccaggcatcgcagacctgcttcacctgctgccaggactcctcccactgccggatcttcctcttggcctcgtccagctgccgcctgacccgggccagctcagctccgtttggacttgcactcgaagaggatggggggccggcactcaggatgggggaggggctgggggagaagctgccggaaacaaagtcccagatgctcccggggacaccgttcaaacctagggggctgtaggatgaggctgcagagcccagtgtgcccggctctgaacgcaggggtggcggctgctggggaggcgtcatggctgaggagcccaccggccctgggaggggctgggacagcgaaccgagcggcgaggtggacgcagaggatggcgagtgtagcgatggtgctctgggcagggagccggggatggcgacaggtgcagagccggccagcgacctgggacctgctgctcccaggtcgtggccgtcttgctcttccaggtccttctctagggatgcaatattcacattgctaagatgcaggtctaacgcagaacctggcggggggcgcacctaagggagggcccgctcctgaccgccgagtaacgagacccgcaccttggcggcgcacggctgccacgcgctggggccgccgccaatgctgactcacggtccgc

SEQ ID NO: 11402 - RNA, 2377 nt, Homo sapiens
  source 1..2377: mol_type = other RNA
ctgaatagctgggactacaggtgcccgctctcacgccaggccaatttttgtatttttactaagacggggttgcaccatgttggccaggctggtcttgaactcctgaccttaggtgatccacccgcctcccaaagtgctgggatcacaggcatgagccaccgcacccagccagaagacagctgcttaaaaaagtaattctaaaagctctgacgtcggatcccctctgctgcgttttttgttagtatcaaactgtctttcagagggttaagggagaaaacaaaacccatgatgctccttcacttgctctccgaggcgcaggcgcacagaaacagcggccacggaccacagaaatgcaggacggagctctcctgctcccacgccacgaggctggaacatcagccccagtgcctggtgcacacacaggctcaggaaaactagctccttccatcaagttaaaaacatctcaatccataatcactctgcttataaatactatttgcacttaattggaaaatgtaaaaatcctaggtcttactactagataaacactcatttcataagtactagtttcagaatatgaaatctaatatatttagcatactatgaattgacaataaactgatatgaaatatttaagttcacagtacacatataaagcttcatattatcgcatattaaaaaaaaacagaaagcagcttagagcaatttataacctctaactaaattcctcggtttacaaagtgctttgaaagaccccagctcccagtggcctagtcacagtagtgtcaggaccacaaactgctgtgatcacagcgccgcgtggatcccggaggcaccaggcccctcagggacaggcaggcgggttctgtgggtttgcatttaaggtttttgaggaaaataccttgaaaccgtcggtaggactagataggtgacaacgtgtgacaggaaaggctgtcaggccaagcgcaggcggggctcccagcctcatgataacgtgtaacaggaagggctcccagcctcggtcctcacgtcggtggcaccagaagcgagtgacgacatgtccgtggtcaggaggagcgctggagccagggtgcccagcaggaggtggctgtccccgctgaggtcaccactgcaggggctggcccttgcagtaggggcactcaggtgcggtggccgcacacggctcacagaggatgtggtgctgacagggccgcaggacagcaccgtgggcccgctcccggcaggccacacactgcttggcgcggagctggaagatcacgccgtccaccgcctccaggtccaggcgcagctgactctgcagcgagtgcagcttcggcaggggaatggtgccgatgtccccacagccccgcagccccggcagtgtggaggctacgcccaggccctccagctcctcctgcagctgcttcacctgtgcctccacctcctccttcttctgcagcgccagctgccggtcgctatcggccacacgggcacgctccttggcctcctgcgcctctcgctgccaggcatcgcagacctgcttcacctgctgccaggactcctcccactgccggatcttcctcttggcctcgtccagctgccgcctgacccgggccagctcagctccgtttggacttgcactcgaagaggatggggggccggcactcaggatgggggaggggctgggggagaagctgccggaaacaaagtcccagatgctcccggggacaccgttcaaaccattgcagtccaacctgggcgacagagcgagactcggtctgcggcgtgggggaacctgtgagcagcaggtcatgtggtttgccaccacagatagggcacaaggttccgtgtgaggcccctcagtcaggacggcatctgggagggagccccacggaggcttcacggcaacgccagcatggagggagccggcactcacctagggggctgtaggatgaggctgcagagcccagtgtgcccggctctgaacgcaggggtggcggctgctggggaggcgtcatggctgaggagcccaccggccctgggaggggctgggacagcgaaccgagcggcgaggtggacgcagaggatggcgagtgtagcgatggtgctctgggcagggagccggggatggcgacaggtgcagagccggccagcgacctgggacctgctgctcccaggtcgtggccgtcttgctcttccaggtccttctctagggatgcaatattcacattgctaagatgcaggtctaacgcagaacctggcggggggcgcacctaagggagggcccgctcctgaccgccgagtaacgagacccgcaccttggcggcgcacggctgccacgcgctggggccgccgccaatgctgactcacggtccgc

SEQ ID NO: 11403 - RNA, 3211 nt, Homo sapiens
  source 1..3211: mol_type = other RNA
ctgaatagctgggactacaggtgcccgctctcacgccaggccaatttttgtatttttactaagacggggttgcaccatgttggccaggctggtcttgaactcctgaccttaggtgatccacccgcctcccaaagtgctgggatcacaggcatgagccaccgcacccagccagaagacagctgcttaaaaaagtaattctaaaagctctgacgtcggatcccctctgctgcgttttttgttagtatcaaactgtctttcagagggttaagggagaaaacaaaacccatgatgctccttcacttgctctccgaggcgcaggcgcacagaaacagcggccacggaccacagaaatgcaggacggagctctcctgctcccacgccacgaggctggaacatcagccccagtgcctggtgcacacacaggctcaggaaaactagctccttccatcaagttaaaaacatctcaatccataatcactctgcttataaatactatttgcacttaattggaaaatgtaaaaatcctaggtcttactactagataaacactcatttcataagtactagtttcagaatatgaaatctaatatatttagcatactatgaattgacaataaactgatatgaaatatttaagttcacagtacacatataaagcttcatattatcgcatattaaaaaaaaacagaaagcagcttagagcaatttataacctctaactaaattcctcggtttacaaagtgctttgaaagaccccagctcccagtggcctagtcacagtagtgtcaggaccacaaactgctgtgatcacagcgccgcgtggatcccggaggcaccaggcccctcagggacaggcaggcgggttctgtgggtttgcatttaaggtttttgaggaaaataccttgaaaccgtcggtaggactagataggtgacaacgtgtgacaggaaaggctgtcaggccaagcgcaggcggggctcccagcctcatgataacgtgtaacaggaagggctcccagcctcggtcctcacgtcggtggcaccagaagcgagtgacgacatgtccgtggtcaggaggagcgctggagccagggtgcccagcaggaggtggctgtccccgctgaggtcaccactgcaggggctggcccttgcagtaggggcactcaggtgcggtggccgcacacggctcacagaggatgtggtgctgacagggccgcaggacagcaccgtgggcccgctcccggcaggccacacactgcttggcgcggagctggaagatcacgccgtccaccgcctccaggtccaggcgcagctgactctgcagcgagtgcagcttcggcaggggaatggtgccgatgtccccacagccccgcagccccggcagtgtggaggctacgcccaggccctccagctcctcctgcagctgcttcacctgtgcctccacctcctccttcttctgcagcgccagctgccggtcgctatcggccacacgggcacgctccttggcctcctgcgcctctcgctgccaggcatcgcagacctgcttcacctgctgccaggactcctcccactgccggatcttcctcttggcctcgtccagctgccgcctgacccgggccagctcagctccgtttggacttgcactcgaagaggatggggggccggcactcaggatgggggaggggctgggggagaagctgccggaaacaaagtcccagatgctcccggggacaccgttcaaacctagggggctgtaggatgaggctgcagagcccagtgtgcccggctctgaacgcaggggtggcggctgctggggaggcgtcatggctgaggagcccaccggccctgggaggggctgggacagcgaaccgagcggcgaggtggacgcagaggatggcgagtgtagcgatggtgctctgggcagggagccggggatggcgacaggtgcagagccggccagcgacctgggacctgctgctcccaggtcgtggccgtcttgctcttccaggtccttctctagggatgcaatattcacattgctaagatgcaggtctaacgcagaaccgaggacggcctccacagtgctgctggcggggccgagcgggagggcacgggcggggggcgcgggcagcgcagtgggggaggagctgccggagccggcgctggacgccaggctggacgccacgctggagctcacgctgggggccggcgggtggaccgctgcaaacacggccaggtggttctgcttgctgtcttgctcgctgcccctagggccaccctcggccggcgagtctctccgcttggcatttcccggctggccgctgcccgtggaggaaggactcgtgaggtggaggtcgtgacagccccattcattcaccatccccaggctcttctcaacgtgtgcaaaggcacagaaggggccgcgcgggcagtacccggtttggcgcatgtcgttgcattttgtagatttgtagatctcgggatggaactgctgctccgtgcgggagtggcaatactggcagccgtcgccgccatcgcagcgtgagggttccccccactcatccccgtgcttcacactggggcagggcgtggacctcctggggacagtgaggccgggcgcccagacagcacggggctgtctcctcgccaactttctgtactggaaccgccgggggttgcgccgcctgtcccggctattgtggtagtgtgggcacgcatagccctggcggcacaggcgtggcggcttcgggcactgctccgtcttgtagctgcccagcacgaagttggcatcttgccaccgggggtcctcgctcaggatcttctcaatcatggcctggctggccaagaccccaggctgcagatccgggaccccttccccgccgcccagctggccgttctgcaaggcttcctgggcctgcagctccctgacgtcacacacgggcggccgcaggtccagggggccgtgcgcgaaggcacagtgcagcccattcttcacgcagtggccacgtgcgtctgtctcgtggatgcaggttcctgttttgtagtaacgcaggtggtacttgcgttctgtgtcccccgtcgtccggtgcaggtagggacacctgtagtgggtcggcttctcagtctgcgggggggacccgctcagcgccgctgccgccgctttcgaaaccgacggcattttcagtcaaaacaatgcagcgcgcatgcgccgcgc

SEQ ID NO: 11404 - RNA, 3443 nt, Homo sapiens
  source 1..3443: mol_type = other RNA
ctgaatagctgggactacaggtgcccgctctcacgccaggccaatttttgtatttttactaagacggggttgcaccatgttggccaggctggtcttgaactcctgaccttaggtgatccacccgcctcccaaagtgctgggatcacaggcatgagccaccgcacccagccagaagacagctgcttaaaaaagtaattctaaaagctctgacgtcggatcccctctgctgcgttttttgttagtatcaaactgtctttcagagggttaagggagaaaacaaaacccatgatgctccttcacttgctctccgaggcgcaggcgcacagaaacagcggccacggaccacagaaatgcaggacggagctctcctgctcccacgccacgaggctggaacatcagccccagtgcctggtgcacacacaggctcaggaaaactagctccttccatcaagttaaaaacatctcaatccataatcactctgcttataaatactatttgcacttaattggaaaatgtaaaaatcctaggtcttactactagataaacactcatttcataagtactagtttcagaatatgaaatctaatatatttagcatactatgaattgacaataaactgatatgaaatatttaagttcacagtacacatataaagcttcatattatcgcatattaaaaaaaaacagaaagcagcttagagcaatttataacctctaactaaattcctcggtttacaaagtgctttgaaagaccccagctcccagtggcctagtcacagtagtgtcaggaccacaaactgctgtgatcacagcgccgcgtggatcccggaggcaccaggcccctcagggacaggcaggcgggttctgtgggtttgcatttaaggtttttgaggaaaataccttgaaaccgtcggtaggactagataggtgacaacgtgtgacaggaaaggctgtcaggccaagcgcaggcggggctcccagcctcatgataacgtgtaacaggaagggctcccagcctcggtcctcacgtcggtggcaccagaagcgagtgacgacatgtccgtggtcaggaggagcgctggagccagggtgcccagcaggaggtggctgtccccgctgaggtcaccactgcaggggctggcccttgcagtaggggcactcaggtgcggtggccgcacacggctcacagaggatgtggtgctgacagggccgcaggacagcaccgtgggcccgctcccggcaggccacacactgcttggcgcggagctggaagatcacgccgtccaccgcctccaggtccaggcgcagctgactctgcagcgagtgcagcttcggcaggggaatggtgccgatgtccccacagccccgcagccccggcagtgtggaggctacgcccaggccctccagctcctcctgcagctgcttcacctgtgcctccacctcctccttcttctgcagcgccagctgccggtcgctatcggccacacgggcacgctccttggcctcctgcgcctctcgctgccaggcatcgcagacctgcttcacctgctgccaggactcctcccactgccggatcttcctcttggcctcgtccagctgccgcctgacccgggccagctcagctccgtttggacttgcactcgaagaggatggggggccggcactcaggatgggggaggggctgggggagaagctgccggaaacaaagtcccagatgctcccggggacaccgttcaaacctagggggctgtaggatgaggctgcagagcccagtgtgcccggctctgaacgcaggggtggcggctgctggggaggcgtcatggctgaggagcccaccggccctgggaggggctgggacagcgaaccgagcggcgaggtggacgcagaggatggcgagtgtagcgatggtgctctgggcagggagccggggatggcgacaggtgcagagccggccagcgacctgggacctgctgctcccaggtcgtggccgtcttgctcttccaggtccttctctagggatgcaatattcacattgctaagatgcaggtctaacgcagaaccgaggacggcctccacagtgctgctggcggggccgagcgggagggcacgggcggggggcgcgggcagcgcagtgggggaggagctgccggagccggcgctggacgccaggctggacgccacgctggagctcacgctgggggccggcgggtggaccgctgcaaacacggccaggtggttctgcttgctgtcttgctcgctgcccctagggccaccctcggccggcgagtctctccgcttggcatttcccggctggccgctgcccgtggaggaaggactcgtgaggtggaggtcgtgacagccccattcattcaccatccccaggctcttctcaacgtgtgcaaaggcacagaaggggccgcgcgggcagtacccggtttggcgcatgtcgttgcattttgtagatttgtagatctcgggatggaactgctgctccgtgcgggagtggcaatactggcagccgtcgccgccatcgcagcgtgagggttccccccactcatccccgtgcttcacactggggcagggcgtggacctcctggggacagtgaggccgggcgcccagacagcacggggctgtctcctcgccaactttctgtactggaaccgccgggggttgcgccgcctgtcccggctattgtggtagtgtgggcacgcatagccctggcggcacaggcgtggcggcttcgggcactgctccgtcttgtagctgcccagcacgaagttggcatcttgccaccgggggtcctcgctcaggatcttctcaatcatggcctggctggccaagaccccaggctgcagatccgggaccccttccccgccgcccagctggccgttctgcaaggcttcctgggcctgcagctccctgacgtcacacacgggcggccgcaggtccagggggccgtgcgcgaaggcacagtgcagcccattcttcacgcagtggccacgtgcgtctgtctcgtggatgcaggttcctgttttgtagtaacgcaggtggtacttgcgttctgtgtcccccgtcgtccggtgcaggtagggacactcgtcgccgtcggggcacacgccggtggcttcgttgtacttggagcagtacacgtcggggctgtagttgaaggtgccgtcgcgcctgcggaggggcctgcggcgccgctggttgaggaagtgccagtggaagcaggtgaacggccggtgctgcgcgcacttgtgctgtgaaaacagggggcactgctccgtcctgaactccttcaggtacctgtagtgggtcggcttctcagtctgcgggggggacccgctcagcgccgctgccgccgctttcgaaaccgacggcattttcagtcaaaacaatgcagcgcgcatgcgccgcgccggcgcccccgcccccggatat

SEQ ID NO: 11405 - RNA, 3338 nt, Homo sapiens
  source 1..3338: mol_type = other RNA
ctgaatagctgggactacaggtgcccgctctcacgccaggccaatttttgtatttttactaagacggggttgcaccatgttggccaggctggtcttgaactcctgaccttaggtgatccacccgcctcccaaagtgctgggatcacaggcatgagccaccgcacccagccagaagacagctgcttaaaaaagtaattctaaaagctctgacgtcggatcccctctgctgcgttttttgttagtatcaaactgtctttcagagggttaagggagaaaacaaaacccatgatgctccttcacttgctctccgaggcgcaggcgcacagaaacagcggccacggaccacagaaatgcaggacggagctctcctgctcccacgccacgaggctggaacatcagccccagtgcctggtgcacacacaggctcaggaaaactagctccttccatcaagttaaaaacatctcaatccataatcactctgcttataaatactatttgcacttaattggaaaatgtaaaaatcctaggtcttactactagataaacactcatttcataagtactagtttcagaatatgaaatctaatatatttagcatactatgaattgacaataaactgatatgaaatatttaagttcacagtacacatataaagcttcatattatcgcatattaaaaaaaaacagaaagcagcttagagcaatttataacctctaactaaattcctcggtttacaaagtgctttgaaagaccccagctcccagtggcctagtcacagtagtgtcaggaccacaaactgctgtgatcacagcgccgcgtggatcccggaggcaccaggcccctcagggacaggcaggcgggttctgtgggtttgcatttaaggtttttgaggaaaataccttgaaaccgtcggtaggactagataggtgacaacgtgtgacaggaaaggctgtcaggccaagcgcaggcggggctcccagcctcatgataacgtgtaacaggaagggctcccagcctcggtcctcacgtcggtggcaccagaagcgagtgacgacatgtccgtggtcaggaggagcgctggagccagggtgcccagcaggaggtggctgtccccgctgaggtcaccactgcaggggctggcccttgcagtaggggcactcaggtgcggtggccgcacacggctcacagaggatgtggtgctgacagggccgcaggacagcaccgtgggcccgctcccggcaggccacacactgcttggcgcggagctggaagatcacgccgtccaccgcctccaggtccaggcgcagctgactctgcagcgagtgcagcttcggcaggggaatggtgccgatgtccccacagccccgcagccccggcagtgtggaggctacgcccaggccctccagctcctcctgcagctgcttcacctgtgcctccacctcctccttcttctgcagcgccagctgccggtcgctatcggccacacgggcacgctccttggcctcctgcgcctctcgctgccaggcatcgcagacctgcttcacctgctgccaggactcctcccactgccggatcttcctcttggcctcgtccagctgccgcctgacccgggccagctcagctccgtttggacttgcactcgaagaggatggggggccggcactcaggatgggggaggggctgggggagaagctgccggaaacaaagtcccagatgctcccggggacaccgttcaaacctagggggctgtaggatgaggctgcagagcccagtgtgcccggctctgaacgcaggggtggcggctgctggggaggcgtcatggctgaggagcccaccggccctgggaggggctgggacagcgaaccgagcggcgaggtggacgcagaggatggcgagtgtagcgatggtgctctgggcagggagccggggatggcgacaggtgcagagccggccagcgacctgggacctgctgctcccaggtcgtggccgtcttgctcttccaggtccttctctagggatgcaatattcacattgctaagatgcaggtctaacgcagaaccgaggacggcctccacagtgctgctggcggggccgagcgggagggcacgggcggggggcgcgggcagcgcagtgggggaggagctgccggagccggcgctggacgccaggctggacgccacgctggagctcacgctgggggccggcgggtggaccgctgcaaacacggccaggtggttctgcttgctgtcttgctcgctgcccctagggccaccctcggccggcgagtctctccgcttggcatttcccggctggccgctgcccgtggaggaaggactcgtgaggtggaggtcgtgacagccccattcattcaccatccccaggctcttctcaacgtgtgcaaaggcacagaaggggccgcgcgggcagtacccggtttggcgcatgtcgttgcattttgtagatttgtagatctcgggatggaactgctgctccgtgcgggagtggcaatactggcagccgtcgccgccatcgcagcgtgagggttccccccactcatccccgtgcttcacactggggcagggcgtggacctgtactggaaccgccgggggttgcgccgcctgtcccggctattgtggtagtgtgggcacgcatagccctggcggcacaggcgtggcggcttcgggcactgctccgtcttgtagctgcccagcacgaagttggcatcttgccaccgggggtcctcgctcaggatcttctcaatcatggcctggctggccaagaccccaggctgcagatccgggaccccttccccgccgcccagctggccgttctgcaaggcttcctgggcctgcagctccctgacgtcacacacgggcggccgcaggtccagggggccgtgcgcgaaggcacagtgcagcccattcttcacgcagtggccacgtgcgtctgtctcgtggatgcaggttcctgttttgtagtaacgcaggtggtacttgcgttctgtgtcccccgtcgtccggtgcaggtagggacactcgtcgccgtcggggcacacgccggtggcttcgttgtacttggagcagtacacgtcggggctgtagttgaaggtgccgtcgcgcctgcggaggggcctgcggcgccgctggttgaggaagtgccagtggaagcaggtgaacggccggtgctgcgcgcacttgtgctgtgaaaacagggggcactgctccgtcctgaactccttcaggtacctgtagtgggtcggcttctcagtctgcgggggggacccgctcagcgccgctgccgccgctttcgaaaccgacggcattttcagtcaaaac

SEQ ID NO: 11406 - RNA, 2324 nt, Homo sapiens
  source 1..2324: mol_type = other RNA
ctgaatagctgggactacaggtgcccgctctcacgccaggccaatttttgtatttttactaagacggggttgcaccatgttggccaggctggtcttgaactcctgaccttaggtgatccacccgcctcccaaagtgctgggatcacaggcatgagccaccgcacccagccagaagacagctgcttaaaaaagtaattctaaaagctctgacgtcggatcccctctgctgcgttttttgttagtatcaaactgtctttcagagggttaagggagaaaacaaaacccatgatgctccttcacttgctctccgaggcgcaggcgcacagaaacagcggccacggaccacagaaatgcaggacggagctctcctgctcccacgccacgaggctggaacatcagccccagtgcctggtgcacacacaggctcaggaaaactagctccttccatcaagttaaaaacatctcaatccataatcactctgcttataaatactatttgcacttaattggaaaatgtaaaaatcctaggtcttactactagataaacactcatttcataagtactagtttcagaatatgaaatctaatatatttagcatactatgaattgacaataaactgatatgaaatatttaagttcacagtacacatataaagcttcatattatcgcatattaaaaaaaaacagaaagcagcttagagcaatttataacctctaactaaattcctcggtttacaaagtgctttgaaagaccccagctcccagtggcctagtcacagtagtgtcaggaccacaaactgctgtgatcacagcgccgcgtggatcccggaggcaccaggcccctcagggacaggcaggcgggttctgtgggtttgcatttaaggtttttgaggaaaataccttgaaaccgtcggtaggactagataggtgacaacgtgtgacaggaaaggctgtcaggccaagcgcaggcggggctcccagcctcatgataacgtgtaacaggaagggctcccagcctcggtcctcacgtcggtggcaccagaagcgagtgacgacatgtccgtggtcaggaggagcgctggagccagggtgcccagcaggaggtggctgtccccgctgaggtcaccactgcaggggctggcccttgcagtaggggcactcaggtgcggtggccgcacacggctcacagaggatgtggtgctgacagggccgcaggacagcaccgtgggcccgctcccggcaggccacacactgcttggcgcggagctggaagatcacgccgtccaccgcctccaggtccaggcgcagctgactctgcagcgagtgcagcttcggcaggggaatggtgccgatgtccccacagccccgcagccccggcagtgtggaggctacgcccaggccctccagctcctcctgcagctgcttcacctgtgcctccacctcctccttcttctgcagcgccagctgccggtcgctatcggccacacgggcacgctccttggcctcctgcgcctctcgctgccaggcatcgcagacctgcttcacctgctgccaggactcctcccactgccggatcttcctcttggcctcgtccagctgccgcctgacccgggccagctcagctccgtttggacttgcactcgaagaggatggggggccggcactcaggatgggggaggggctgggggagaagctgccggaaacaaagtcccagatgctcccggggacaccgttcaaacctagggggctgtaggatgaggctgcagagcccagtgtgcccggctctgaacgcaggggtggcggctgctggggaggcgtcatggctgaggagcccaccggccctgggaggggctgggacagcgaaccgagcggcgaggtggacgcagaggatggcgagtgtagcgatggtgctctgggcagggagccggggatggcgacaggtgcagagccggccagcgacctgggacctgctgctcccaggtcgtggccgtcttgctcttccaggtccttctctagggatgcaatattcacattgctaagatgcaggtctaacgcagaacctcactgtttcaaggttagacccagatcttctgaaacattctcaaagaaagagctgacccttgtgcagaggcaaaatctaggtgaggctggtcacctaagcgagtacagctgggtcaggccaggctgcctcagccccgggcgttaggaaaccaccggccccgctgagtcaccgcgacacagcccggctctgccgtgacacagcacattcaaggcgccgcggtcccccggggtcagggacacgcgaggacaagctacagactgc

SEQ ID NO: 11407 - RNA, 2181 nt, Homo sapiens
  source 1..2181: mol_type = other RNA
ctgaatagctgggactacaggtgcccgctctcacgccaggccaatttttgtatttttactaagacggggttgcaccatgttggccaggctggtcttgaactcctgaccttaggtgatccacccgcctcccaaagtgctgggatcacaggcatgagccaccgcacccagccagaagacagctgcttaaaaaagtaattctaaaagctctgacgtcggatcccctctgctgcgttttttgttagtatcaaactgtctttcagagggttaagggagaaaacaaaacccatgatgctccttcacttgctctccgaggcgcaggcgcacagaaacagcggccacggaccacagaaatgcaggacggagctctcctgctcccacgccacgaggctggaacatcagccccagtgcctggtgcacacacaggctcaggaaaactagctccttccatcaagttaaaaacatctcaatccataatcactctgcttataaatactatttgcacttaattggaaaatgtaaaaatcctaggtcttactactagataaacactcatttcataagtactagtttcagaatatgaaatctaatatatttagcatactatgaattgacaataaactgatatgaaatatttaagttcacagtacacatataaagcttcatattatcgcatattaaaaaaaaacagaaagcagcttagagcaatttataacctctaactaaattcctcggtttacaaagtgctttgaaagaccccagctcccagtggcctagtcacagtagtgtcaggaccacaaactgctgtgatcacagcgccgcgtggatcccggaggcaccaggcccctcagggacaggcaggcgggttctgtgggtttgcatttaaggtttttgaggaaaataccttgaaaccgtcggtaggactagataggtgacaacgtgtgacaggaaaggctgtcaggccaagcgcaggcggggctcccagcctcatgataacgtgtaacaggaagggctcccagcctcggtcctcacgtcggtggcaccagaagcgagtgacgacatgtccgtggtcaggaggagcgctggagccagggtgcccagcaggaggtggctgtccccgctgaggtcaccactgcaggggctggcccttgcagtaggggcactcaggtgcggtggccgcacacggctcacagaggatgtggtgctgacagggccgcaggacagcaccgtgggcccgctcccggcaggccacacactgcttggcgcggagctggaagatcacgccgtccaccgcctccaggtccaggcgcagctgactctgcagcgagtgcagcttcggcaggggaatggtgccgatgtccccacagccccgcagccccggcagtgtggaggctacgcccaggccctccagctcctcctgcagctgcttcacctgtgcctccacctcctccttcttctgcagcgccagctgccggtcgctatcggccacacgggcacgctccttggcctcctgcgcctctcgctgccaggcatcgcagacctgcttcacctgctgccaggactcctcccactgccggatcttcctcttggcctcgtccagctgccgcctgacccgggccagctcagctccgtttggacttgcactcgaagaggatggggggccggcactcaggatgggggaggggctgggggagaagctgccggaaacaaagtcccagatgctcccggggacaccgttcaaacctagggggctgtaggatgaggctgcagagcccagtgtgcccggctctgaacgcaggggtggcggctgctggggaggcgtcatggctgaggagcccaccggccctgggaggggctgggacagcgaaccgagcggcgaggtggacgcagaggatggcgagtgtagcgatggtgctctgggcagggagccggggatggcgacaggtgcagagccggccagcgacctgggacctgctgctcccaggtcgtggccgtcttgctcttccaggtccttctctagggatgcaatattcacattgctaagatgcaggtctaacgcagaacctggcggggggcgcacctaagggagggcccgctcctgaccgccgagtaacgagacccgcaccttggcggcgcacggctgccacgcgctggggccgccgccaatgctgactcacggtccgc

SEQ ID NO: 11408 - RNA, 1953 nt, Homo sapiens
  source 1..1953: mol_type = other RNA
ctgaatagctgggactacaggtgcccgctctcacgccaggccaatttttgtatttttactaagacggggttgcaccatgttggccaggctggtcttgaactcctgaccttaggtgatccacccgcctcccaaagtgctgggatcacaggcatgagccaccgcacccagccagaagacagctgcttaaaaaagtaattctaaaagctctgacgtcggatcccctctgctgcgttttttgttagtatcaaactgtctttcagagggttaagggagaaaacaaaacccatgatgctccttcacttgctctccgaggcgcaggcgcacagaaacagcggccacggaccacagaaatgcaggacggagctctcctgctcccacgccacgaggctggaacatcagccccagtgcctggtgcacacacaggctcaggaaaactagctccttccatcaagttaaaaacatctcaatccataatcactctgcttataaatactatttgcacttaattggaaaatgtaaaaatcctaggtcttactactagataaacactcatttcataagtactagtttcagaatatgaaatctaatatatttagcatactatgaattgacaataaactgatatgaaatatttaagttcacagtacacatataaagcttcatattatcgcatattaaaaaaaaacagaaagcagcttagagcaatttataacctctaactaaattcctcggtttacaaagtgctttgaaagaccccagctcccagtggcctagtcacagtagtgtcaggaccacaaactgctgtgatcacagcgccgcgtggatcccggaggcaccaggcccctcagggacaggcaggcgggttctgtgggtttgcatttaaggtttttgaggaaaataccttgaaaccgtcggtaggactagataggtgacaacgtgtgacaggaaaggctgtcaggccaagcgcaggcggggctcccagcctcatgataacgtgtaacaggaagggctcccagcctcggtcctcacgtcggtggcaccagaagcgagtgacgacatgtccgtggtcaggaggagcgctggagccagggtgcccagcaggaggtggctgtccccgctgaggtcaccactgcaggggctggcccttgcagtaggggcactcaggtgcggtggccgcacacggctcacagaggatgtggtgctgacagggccgcaggacagcaccgtgggcccgctcccggcaggccacacactgcttggcgcggagctggaagatcacgccgtccaccgcctccaggtccaggcgcagctgactctgcagcgagtgcagcttcggcaggggaatggtgccgatgtccccacagccccgcagccccggcagtgtggaggctacgcccaggccctccagctcctcctgcagctgcttcacctgtgcctccacctcctccttcttctgcagcgccagctgccggtcgctatcggccacacgggcacgctccttggcctcctgcgcctctcgctgccaggcatcgcagacctgcttcacctgctgccaggactcctcccactgccggatcttcctcttggcctcgtccagctgccgcctgacccgggccagctcagctccgtttggacttgcactcgaagaggatggggggccggcactcaggatgggggaggggctgggggagaagctgccggaaacaaagtcccagatgctcccggggacaccgttcaaacctgctgctcccaggtcgtggccgtcttgctcttccaggtccttctctagggatgcaatattcacattgctaagatgcaggtctaacgcagaacctggcggggggcgcacctaagggagggcccgctcctgaccgccgagtaacgagacccgcaccttggcggcgcacggctgccacgcgctggggccgccgccaatgctgactcacggtccgc

SEQ ID NO: 11409 - RNA, 1201 nt, Homo sapiens
  source 1..1201: mol_type = other RNA
ctgaatagctgggactacaggtgcccgtcaccatgcccggctaattttttattttttgtatttttagtagagacggggtttcaccgtgttagccaggatggtcttgatctcctgaccttgtgatccgccctcctcagccttccaaagtgctaggattacaggcatgagctgctgtgctggccctcagaggttaattttcaatcttcactcgaccactcgtgagctaaatgagttccccttttctgcagtctatttttccatacatccaatttatttaacaaggtggagcctcatctgaagcatttcctcaccaggcttgaagagggccatttttccattagagcatcaggctgacttattggtatcggacgaagactcctctccacgagtcaagtactggatttttttcctcttgagttcctcctggaggctctctcttaggcttatttcccgctctgttgcagcatatcccatttctttcatctcttgctcactttctatctcactggacagagcagttatttccttctgttgtctccacaagaagtaactggctccggcgagaagcagcagcaagataggcagggtccctgccagggctgcgatccagggctgggcgctcctgaagaaggggtctgcaaccttcagctccaccagggctttttcatagaagtcaccatcttggaaataacacaagtactttccactgtcagaggctgtgacgttgtgtattcggagagcagccttccctgcagtgatgccatcccgcagaatcgaagttctccctcgatacggtgcactctgcctgtcttccacttcctttccatctgcatacacgttcaccacctgccttaggctggaacttacccacttcagctccatggtctctgcactcatggtcgggaacaggtgacagggcagatcagcgtcttcacccaccatggccaggatgggcccagagggtccaagcacagaaaactgagctctgccaaaaatgtctgtccttgagtgtctttacctttgggttccagtatggaaaaccatcccttggtattcccattggagaatcagagcccacagaataaagacggtcaatcaataattctccattctttctattatggcttagcctctcatccggaagaaaggaaaaagagaaagcaaatattgtcttctcaccatgagaaacagtaagagtcgc

SEQ ID NO: 11410 - RNA, 1182 nt, Homo sapiens
  source 1..1182: mol_type = other RNA
ctgaatagctgggactacaggtgcccgtcaccatgcccggctaattttttattttttgtatttttagtagagacggggtttcaccgtgttagccaggatggtcttgatctcctgaccttgtgatccgccctcctcagccttccaaagtgctaggattacaggcatgagctgctgtgctggccctcagaggttaattttcaatcttcactcgaccactcgtgagctaaatgagttccccttttctgcagtctatttttccatacatccaatttatttaacaaggtggagcctcatctgaagcatttcctcaccaggcttgaagagggccatttttccattagagcatcaggctgacttattggtatcggacgaagactcctctccacgagtcaagtactggatttttttcctcttgagttcctcctggaggctctctcttaggcttatttcccgctctgttgcagcatatcccatttctttcatctcttgctcactttctatctcactggacagagcagttatttccttctgttgtctccacaagaagtaactggctccggcgagaagcagcagcaagataggcagggtccctgccagggctgcgatccagggctgggcgctcctgaagaaggggtctgcaaccttcagctccaccagggctttttcatagaagtcaccatcttggaaataacacaagtactttccactgtcagaggctgtgacgttgtgtattcggagagcagccttccctgcagtgatgccatcccgcagaatcgaagttctccctcgatacggtgcactctgcctgtcttccacttcctttccatctgcatacacgttcaccacctgccttaggctggaacttacccacttcagctccatggtctctgcactcatggtcgggaacaggtgacagggcagatcagcgtcttcacccaccatggccaggatgggcccagagggtccaagcacagaaaactgagctgagcaaggagtgagcagctggaccaagaggagggagacatgaaagttgagcagaaggaaagccagggaacttgccattttcatctatgctctgccaaaaatgtctgtccttgagtgtctttacctttgggttccagtatggaaaaccatcatgagaaacagtaagagtcgctctttggaagaattagttttttgatt

SEQ ID NO: 11411 - RNA, 1588 nt, Homo sapiens
  source 1..1588: mol_type = other RNA
ctgaatagctgggactacaggtgcccgtcaccatgcccggctaattttttattttttgtatttttagtagagacggggtttcaccgtgttagccaggatggtcttgatctcctgaccttgtgatccgccctcctcagccttccaaagtgctaggattacaggcatgagctgctgtgctggccctcagaggttaattttcaatcttcactcgaccactcgtgagctaaatgagttccccttttctgcagtctatttttccatacatccaatttatttaacaaggtggagcctcatctgaagcatttcctcaccaggcttgaagagggccatttttccattagagcatcaggctgacttattggtatcggacgaagactcctctccacgagtcaagtactggatttttttcctcttgagttcctcctggaggctctctcttaggcttatttcccgctctgttgcagcatatcccatttctttcatctcttgctcactttctatctcactggacagagcagttatttccttctgttgtctccacaagaagtaactggctccggcgagaagcagcagcaagataggcagggtccctgccagggctgcgatccagggctgggcgctcctgaagaaggggtctgcgaaggggagagctgcgatggaaatgctggctgtcttttccaggccgaggagggaatttctgatgatgcaggatacaccctccccggagccgcctctcatgatcacagatgctgctacttcatataggcccactccatctgcaaccacaggtgcttccacagctgggatgttctctcccttggcgttgctccactgtatttggggttgggggtaccagccggtggacctgcactccagatggatccctccatcctcataacccttcacttcgacgtgaagattagaacccagtgctgcaaccttcagctccaccagggctttttcatagaagtcaccatcttggaaataacacaagtactttccactgtcagaggctgtgacgttgtgtattcggagagcagccttccctgcagtgatgccatcccgcagaatcgaagttctccctcgatacggtgcactctgcctgtcttccacttcctttccatctgcatacacgttcaccacctgccttaggctggaacttacccacttcagctccatggtctctgcactcatggtcgggaacaggtgacagggcagatcagcgtcttcacccaccatggccaggatgggcccagagggtccaagcacagaaaactgagctgagcaaggagtgagcagctggaccaagaggagggagacatgaaagttgagcagaaggaaagccagggaacttgccattttcatctatgctctgccaaaaatgtctgtccttgagtgtctttacctttgggttccagtatggaaaaccatcccttggtattcccattggagaatcagagcccacagaataaagacggtcaatcaataattctccattctttctattatggcttagcctctcatccggaagaaaggaaaaagagaaagcaaatattgtcttctcaccatgagaaacagtaagagtcgc

SEQ ID NO: 11412 - RNA, 1420 nt, Homo sapiens
  source 1..1420: mol_type = other RNA
ctgaatagctgggactacaggtgcccgtcaccatgcccggctaattttttattttttgtatttttagtagagacggggtttcaccgtgttagccaggatggtcttgatctcctgaccttgtgatccgccctcctcagccttccaaagtgctaggattacaggcatgagctgctgtgctggccctcagaggttaattttcaatcttcactcgaccactcgtgagctaaatgagttccccttttctgcagtctatttttccatacatccaatttatttaacaaggtggagcctcatctgaagcatttcctcaccaggcttgaagagggccatttttccattagagcatcaggctgacttattggtatcggacgaagactcctctccacgagtcaagtactggatttttttcctcttgagttcctcctggaggctctctcttaggcttatttcccgctctgttgcagcatatcccatttctttcatctcttgctcactttctatctcactggacagagcagttatttccttctgttgtctccacaagaagtaactggctccggcgagaagcagcagcaagataggcagggtccctgccagggctgcgatccagggctgggcgctcctgaagaaggggtctgcgatggaaatgctggctgtcttttccaggccgaggagggaatttctgatgatgcaggatacaccctccccggagccgcctctcatgatcacagatgctgctacttcatataggcccactccatctgcaaccacaggtgcttccacagctgggatgttctctcccttggcgttgctccactgtatttggggttgggggtaccagccggtggacctgcactccagatggatccctccatcctcataacccttcacttcgacgtgaagattagaacccagtgctgcaaccttcagctccaccagggctttttcatagaagtcaccatcttggaaataacacaagtactttccactgtcagaggctgtgacgttgtgtattcggagagcagccttccctgcagtgatgccatcccgcagaatcgaagttctccctcgatacggtgcactctgcctgtcttccacttcctttccatctgcatacacgttcaccacctgccttaggctggaacttacccacttcagctccatggtctctgcactcatggtcgggaacaggtgacagggcagatcagcgtcttcacccaccatggccaggatgggcccagagggtccaagcacagaaaactgagcccttggtattcccattggagaatcagagcccacagaataaagacggtcaatcaataattctccattctttctattatggcttagcctctcatccggaagaaaggaaaaagagaaagcaaatattgtcttctcaccatgagaaacagtaagagtc

SEQ ID NO: 11413 - RNA, 1481 nt, Homo sapiens
  source 1..1481: mol_type = other RNA
ctgaatagctgggactacaggtgcccgtcaccatgcccggctaattttttattttttgtatttttagtagagacggggtttcaccgtgttagccaggatggtcttgatctcctgaccttgtgatccgccctcctcagccttccaaagtgctaggattacaggcatgagctgctgtgctggccctcagaggttaattttcaatcttcactcgaccactcgtgagctaaatgagttccccttttctgcagtctatttttccatacatccaatttatttaacaaggtggagcctcatctgaagcatttcctcaccaggcttgaagagggccatttttccattagagcatcaggctgacttattggtatcggacgaagactcctctccacgagtcaagtactggatttttttcctcttgagttcctcctggaggctctctcttaggcttatttcccgctctgttgcagcatatcccatttctttcatctcttgctcactttctatctcactggacagagcagttatttccttctgttgtctccacaagaagtaactggctccggcgagaagcagcagcaagataggcagggtccctgccagggctgcgatccagggctgggcgctcctgaagaaggggtctgcgatggaaatgctggctgtcttttccaggccgaggagggaatttctgatgatgcaggatacaccctccccggagccgcctctcatgatcacagatgctgctacttcatataggcccactccatctgcaaccacaggtgcttccacagctgggatgttctctcccttggcgttgctccactgtatttggggttgggggtaccagccggtggacctgcactccagatggatccctccatcctcataacccttcacttcgacgtgaagattagaacccagtgctgcaaccttcagctccaccagggctttttcatagaagtcaccatcttggaaataacacaagtactttccactgtcagaggctgtgacgttgtgtattcggagagcagccttccctgcagtgatgccatcccgcagaatcgaagttctccctcgatacggtgcactctgcctgtcttccacttcctttccatctgcatacacgttcaccacctgccttaggctggaacttacccacttcagctccatggtctctgcactcatggtcgggaacaggtgacagggcagatcagcgtcttcacccaccatggccaggatgggcccagagggtccaagcacagaaaactgagctctgccaaaaatgtctgtccttgagtgtctttacctttgggttccagtatggaaaaccatcccttggtattcccattggagaatcagagcccacagaataaagacggtcaatcaataattctccattctttctattatggcttagcctctcatccggaagaaaggaaaaagagaaagcaaatattgtcttctcaccatgagaaacagtaagagtc

SEQ ID NO: 11414 - RNA, 1464 nt, Homo sapiens
  source 1..1464: mol_type = other RNA
ctgaatagctgggactacaggtgcccgtcaccatgcccggctaattttttattttttgtatttttagtagagacggggtttcaccgtgttagccaggatggtcttgatctcctgaccttgtgatccgccctcctcagccttccaaagtgctaggattacaggcatgagctgctgtgctggccctcagaggttaattttcaatcttcactcgaccactcgtgagctaaatgagttccccttttctgcagtctatttttccatacatccaatttatttaacaaggtggagcctcatctgaagcatttcctcaccaggcttgaagagggccatttttccattagagcatcaggctgacttattggtatcggacgaagactcctctccacgagtcaagtactggatttttttcctcttgagttcctcctggaggctctctcttaggcttatttcccgctctgttgcagcatatcccatttctttcatctcttgctcactttctatctcactggacagagcagttatttccttctgttgtctccacaagaagtaactggctccggcgagaagcagcagcaagataggcagggtccctgccagggctgcgatccagggctgggcgctcctgaagaaggggtctgcgatggaaatgctggctgtcttttccaggccgaggagggaatttctgatgatgcaggatacaccctccccggagccgcctctcatgatcacagatgctgctacttcatataggcccactccatctgcaaccacaggtgcttccacagctgggatgttctctcccttggcgttgctccactgtatttggggttgggggtaccagccggtggacctgcactccagatggatccctccatcctcataacccttcacttcgacgtgaagattagaacccagtgctgcaaccttcagctccaccagggctttttcatagaagtcaccatcttggaaataacacaagtactttccactgtcagaggctgtgacgttgtgtattcggagagcagccttccctgcagtgatgccatcccgcagaatcgaagttctccctcgatacggtgcactctgcctgtcttccacttcctttccatctgcatacacgttcaccacctgccttaggctggaacttacccacttcagctccatggtctctgcactcatggtcgggaacaggtgacagggcagatcagcgtcttcacccaccatggccaggatgggcccagagggtccaagcacagaaaactgagctgagcaaggagtgagcagctggaccaagaggagggagacatgaaagttgagcagaaggaaagccagggaacttgccattttcatctatgctctgccaaaaatgtctgtccttgagtgtctttacctttgggttccagtatggaaaaccatcatgagaaacagtaagagtcgctctttggaagaattagttttttgatt

SEQ ID NO: 11415 - RNA, 1571 nt, Homo sapiens
  source 1..1571: mol_type = other RNA
ctgaatagctgggactacaggtgcccgtcaccatgcccggctaattttttattttttgtatttttagtagagacggggtttcaccgtgttagccaggatggtcttgatctcctgaccttgtgatccgccctcctcagccttccaaagtgctaggattacaggcatgagctgctgtgctggccctcagaggttaattttcaatcttcactcgaccactcgtgagctaaatgagttccccttttctgcagtctatttttccatacatccaatttatttaacaaggtggagcctcatctgaagcatttcctcaccaggcttgaagagggccatttttccattagagcatcaggctgacttattggtatcggacgaagactcctctccacgagtcaagtactggatttttttcctcttgagttcctcctggaggctctctcttaggcttatttcccgctctgttgcagcatatcccatttctttcatctcttgctcactttctatctcactggacagagcagttatttccttctgttgtctccacaagaagtaactggctccggcgagaagcagcagcaagataggcagggtccctgccagggctgcgatccagggctgggcgctcctgaagaaggggtctgcgatggaaatgctggctgtcttttccaggccgaggagggaatttctgatgatgcaggatacaccctccccggagccgcctctcatgatcacagatgctgctacttcatataggcccactccatctgcaaccacaggtgcttccacagctgggatgttctctcccttggcgttgctccactgtatttggggttgggggtaccagccggtggacctgcactccagatggatccctccatcctcataacccttcacttcgacgtgaagattagaacccagtgctgcaaccttcagctccaccagggctttttcatagaagtcaccatcttggaaataacacaagtactttccactgtcagaggctgtgacgttgtgtattcggagagcagccttccctgcagtgatgccatcccgcagaatcgaagttctccctcgatacggtgcactctgcctgtcttccacttcctttccatctgcatacacgttcaccacctgccttaggctggaacttacccacttcagctccatggtctctgcactcatggtcgggaacaggtgacagggcagatcagcgtcttcacccaccatggccaggatgggcccagagggtccaagcacagaaaactgagctgagcaaggagtgagcagctggaccaagaggagggagacatgaaagttgagcagaaggaaagccagggaacttgccattttcatctatgctctgccaaaaatgtctgtccttgagtgtctttacctttgggttccagtatggaaaaccatcccttggtattcccattggagaatcagagcccacagaataaagacggtcaatcaataattctccattctttctattatggcttagcctctcatccggaagaaaggaaaaagagaaagcaaatattgtcttctcaccatgagaaacagtaagagtc

SEQ ID NO: 11416 - RNA, 1588 nt, Homo sapiens
  source 1..1588: mol_type = other RNA
ctgaatagctgggactacaggtgcccgtcaccatgcccggctaattttttattttttgtatttttagtagagacggggtttcaccgtgttagccaggatggtcttgatctcctgaccttgtgatccgccctcctcagccttccaaagtgctaggattacaggcatgagctgctgtgctggccctcagaggttaattttcaatcttcactcgaccactcgtgagctaaatgagttccccttttctgcagtctatttttccatacatccaatttatttaacaaggtggagcctcatctgaagcatttcctcaccaggcttgaagagggccatttttccattagagcatcaggctgacttattggtatcggacgaagactcctctccacgagtcaagtactggatttttttcctcttgagttcctcctggaggctctctcttaggcttatttcccgctctgttgcagcatatcccatttctttcatctcttgctcactttctatctcactggacagagcagttatttccttctgttgtctccacaagaagtaactggctccggcgagaagcagcagcaagataggcagggtccctgccagggctgcgatccagggctgggcgctcctgaagaaggggtctgcgatggaaatgctggctgtcttttccaggccgaggagggaatttctgatgatgcaggatacaccctccccggagccgcctctcatgatcacagatgctgctacttcatataggcccactccatctgcaaccacaggtgcttccacagctgggatgttctctcccttggcgttgctccactgtatttggggttgggggtaccagccggtggacctgcactccagatggatccctccatcctcataacccttcacttcgacgtgaagattagaacccagtgctgcaaccttcagctccaccagggctttttcatagaagtcaccatcttggaaataacacaagtactttccactgtcagaggctgtgacgttgtgtattcggagagcagccttccctgcagtgatgccatcccgcagaatcgaagttctccctcgatacggtgcactctgcctgtcttccacttcctttccatctgcatacacgttcaccacctgccttaggctggaacttacccacttcagctccatggtctctgcactcatggtcgggaacaggtgacagggcagatcagcgtcttcacccaccatggccaggatgggcccagagggtccaagcacagaaaactgagctgagcaaggagtgagcagctggaccaagaggagggagacatgaaagttgagcagaaggaaagccagggaacttgccattttcatctatgctctgccaaaaatgtctgtccttgagtgtctttacctttgggttccagtatggaaaaccatctgtaaaaataatatcccttggtattcccattggagaatcagagcccacagaataaagacggtcaatcaataattctccattctttctattatggcttagcctctcatccggaagaaaggaaaaagagaaagcaaatattgtcttctcaccatgagaaacagtaagagtcgc

SEQ ID NO: 11417 - RNA, 1295 nt, Homo sapiens
  source 1..1295: mol_type = other RNA
ctgaatagctgggactacaggtgcccgtcaccatgcccggctaattttttattttttgtatttttagtagagacggggtttcaccgtgttagccaggatggtcttgatctcctgaccttgtgatccgccctcctcagccttccaaagtgctaggattacaggcatgagctgctgtgctggccctcagaggttaattttcaatcttcactcgaccactcgtgagctaaatgagttccccttttctgcagtctatttttccatacatccaatttatttaacaaggtggagcctcatctgaagcatttcctcaccaggcttgaagagggccatttttccattagagcatcaggctgacttattggtatcggacgaagactcctctccacgagtcaagtactggatttttttcctcttgagttcctcctggaggctctctgcgatggaaatgctggctgtcttttccaggccgaggagggaatttctgatgatgcaggatacaccctccccggagccgcctctcatgatcacagatgctgctacttcatataggcccactccatctgcaaccacaggtgcttccacagctgggatgttctctcccttggcgttgctccactgtatttggggttgggggtaccagccggtggacctgcactccagatggatccctccatcctcataacccttcacttcgacgtgaagattagaacccagtgctgcaaccttcagctccaccagggctttttcatagaagtcaccatcttggaaataacacaagtactttccactgtcagaggctgtgacgttgtgtattcggagagcagccttccctgcagtgatgccatcccgcagaatcgaagttctccctcgatacggtgcactctgcctgtcttccacttcctttccatctgcatacacgttcaccacctgccttaggctggaacttacccacttcagctccatggtctctgcactcatggtcgggaacaggtgacagggcagatcagcgtcttcacccaccatggccaggatgggcccagagggtccaagcacagaaaactgagctctgccaaaaatgtctgtccttgagtgtctttacctttgggttccagtatggaaaaccatcccttggtattcccattggagaatcagagcccacagaataaagacggtcaatcaataattctccattctttctattatggcttagcctctcatccggaagaaaggaaaaagagaaagcaaatattgtcttctcaccatgagaaacagtaagagtcgctctttggaagaat

SEQ ID NO: 11418 - RNA, 1372 nt, Homo sapiens
  source 1..1372: mol_type = other RNA
ctgaatagctgggactacaggtgcccgtcaccatgcccggctaattttttattttttgtatttttagtagagacggggtttcaccgtgttagccaggatggtcttgatctcctgaccttgtgatccgccctcctcagccttccaaagtgctaggattacaggcatgagctgctgtgctggccctcagaggttaattttcaatcttcactcgaccactcgtgagctaaatgagttccccttttctgcagtctatttttccatacatccaatttatttaacaaggtggagcctcatctgaagcatttcctcaccaggcttgaagagggccatttttccattagagcatcaggctgacttattggtatcggacgaagactcctctccacgagtcaagtactggatttttttcctcttgagttcctcctggaggctctctgcgatggaaatgctggctgtcttttccaggccgaggagggaatttctgatgatgcaggatacaccctccccggagccgcctctcatgatcacagatgctgctacttcatataggcccactccatctgcaaccacaggtgcttccacagctgggatgttctctcccttggcgttgctccactgtatttggggttgggggtaccagccggtggacctgcactccagatggatccctccatcctcataacccttcacttcgacgtgaagattagaacccagtgctgcaaccttcagctccaccagggctttttcatagaagtcaccatcttggaaataacacaagtactttccactgtcagaggctgtgacgttgtgtattcggagagcagccttccctgcagtgatgccatcccgcagaatcgaagttctccctcgatacggtgcactctgcctgtcttccacttcctttccatctgcatacacgttcaccacctgccttaggctggaacttacccacttcagctccatggtctctgcactcatggtcgggaacaggtgacagggcagatcagcgtcttcacccaccatggccaggatgggcccagagggtccaagcacagaaaactgagctgagcaaggagtgagcagctggaccaagaggagggagacatgaaagttgagcagaaggaaagccagggaacttgccattttcatctatgctctgccaaaaatgtctgtccttgagtgtctttacctttgggttccagtatggaaaaccatcccttggtattcccattggagaatcagagcccacagaataaagacggtcaatcaataattctccattctttctattatggcttagcctctcatccggaagaaaggaaaaagagaaagcaaatattgtcttctcaccatgagaaacagtaagagtcgc

SEQ ID NO: 11419 - RNA, 1863 nt, Homo sapiens
  source 1..1863: mol_type = other RNA
ctgaatagctgggactacaggtgcccgtcaccatgcccggctaattttttattttttgtatttttagtagagacggggtttcaccgtgttagccaggatggtcttgatctcctgaccttgtgatccgccctcctcagccttccaaagtgctaggattacaggcatgagctgctgtgctggccctcagaggttaattttcaatcttcactcgaccactcgtgagctaaatgagttccccttttctgcagtctatttttccatacatccaatttatttaacaaggtggagcctcatctgaagcatttcctcacctgaaaaatggggataaacatatgaatctctagcgctgtagaaggcaatcatattatttactcagcccacagcaggccatgaaggaagctcctcatcttcctgatagctgcaaggccgtctctgtgctgggctctgtgtggggccttatatgccctagattcactctccagccttcagctttctccaccctcttctggaccccaggaatctgtcctctatggacagtgccactgggctcccttgtcctctggtttgctgctgtgtttggccaatgggaggcccaggcttgaagagggccatttttccattagagcatcaggctgacttattggtatcggacgaagactcctctccacgagtcaagtactggatttttttcctcttgagttcctcctggaggctctctcttaggcttatttcccgctctgttgcagcatatcccatttctttcatctcttgctcactttctatctcactggacagagcagttatttccttctgttgtctccacaagaagtaactggctccggcgagaagcagcagcaagataggcagggtccctgccagggctgcgatccagggctgggcgctcctgaagaaggggtctgcgatggaaatgctggctgtcttttccaggccgaggagggaatttctgatgatgcaggatacaccctccccggagccgcctctcatgatcacagatgctgctacttcatataggcccactccatctgcaaccacaggtgcttccacagctgggatgttctctcccttggcgttgctccactgtatttggggttgggggtaccagccggtggacctgcactccagatggatccctccatcctcataacccttcacttcgacgtgaagattagaacccagtgctgcaaccttcagctccaccagggctttttcatagaagtcaccatcttggaaataacacaagtactttccactgtcagaggctgtgacgttgtgtattcggagagcagccttccctgcagtgatgccatcccgcagaatcgaagttctccctcgatacggtgcactctgcctgtcttccacttcctttccatctgcatacacgttcaccacctgccttaggctggaacttacccacttcagctccatggtctctgcactcatggtcgggaacaggtgacagggcagatcagcgtcttcacccaccatggccaggatgggcccagagggtccaagcacagaaaactgagctgagcaaggagtgagcagctggaccaagaggagggagacatgaaagttgagcagaaggaaagccagggaacttgccattttcatctctgccaaaaatgtctgtccttgagtgtctttacctttgggttccagtatggaaaaccatctgtaaaaataatatcccttggtattcccattggagaatcagagcccacagaataaagacggtcaatcaataattctccattctttctattatggcttagcctctcatccggaagaaaggaaaaagagaaagcaaatattgtcttctcaccatgagaaacagtaagagtc

SEQ ID NO: 11420 - RNA, 1893 nt, Homo sapiens
  source 1..1893: mol_type = other RNA
ctgaatagctgggactacaggtgccctccaccactcccagctaatttagtagagacagagaaccctgtctctactaaaaatacacccacccagcctaattttcgtatttttagtggagacggggtttcaccatgttggccaggctggtctcgaactcctgacctcaagtgatccacccacctcagcctcccaaagtgctgggattaaaggtgtgagccactgcgcccggccacactcaaatgtctgttaaaataatgaatgcaaacagctcttggccttgaacataccagtgtgcgcttgagctaaactcagtcactcactgcaccagggcctgctagttccctccaacttagaaggggaaaaaatgacacaaagccctaattagcaagaatggccaaggaggttgggcgtggtggctcctgcctgtaatgccagcaatttgggatgccaaggtgggaggactgcttgagcccaggagttcaggaccagcctgagcaacatagtgagaccccatctctataaaagaataaaaacattagccgggcatgggggcatgtgcctgtagtccccgtctctagttaagtactttagtctcctcgggaggctgaggtgggaggatcgcttgagcctgggaggttgaggctgcagtgagccgtgatctcaccactgcattccagcctgggtggcagagtgagaccctgtctcaagagaaaacaagacaaacaagaatggctcagggattgagggctttaagttcattttctggttggctgtgaaaagcatccccttttgggtcccaagcccctgctgacagtcactctatatgtcccatttcctgcttgcctctggcggttcagactcatgcaggccccagacgcctctgtgtgcttagtatgaggcggcgggctgcagggcctgtggaggaagggcagttatccccaggaaaccctgggagtgtctatggtgtgtgtagtcggttaaacctggcaggtccaagtgcggcagggccttgctagaatgctccctgtgccccgtgcacccaaaggggtcatactctgtgtctagtttacaggagaacgccatcggggatgacggagcgtgtgcggtggcccgtgcactgaaggtcaacacagccctcactgctctctagtaagtcctagatgtgcgcagcagtcaggaaaccggtcccttcgccatcctttcacgttagaggtctttttttttttttttttcctcgagacaagagtcttgctctgccacccaggctggagtgcagtgacataatctcagctaactgtaacctccacctcctgggttcaagtgattctcaagcctcagcctcccatacagtagttgggataacaggcgtgcaccaccacacccagcctaatttttgtatttttagtagagacggggtttcaccatattggccaggctggtctcaaactcctgacttcaggtgatctgcccacctcagcctcccaaagtgctgggattacaggtgtgagccaccacacctggcctggacgttatttttgtttacaagtcaaggaaggtgtgtttgattttcctaatataggaaatatgatattagcagttgggggctcaaacacctagagagtagtaatgaggaggtacagggagcattctccccgagcccttccagggacagcctctatttctcatctccttagcatccagatctctgtcttaggcaacagacagtgtaggtaggagatggagtgcctagacacagcgctggccaaccattctcagtgctgtttctccactttccatcctgagtcaaggggtggtgaaagggaacggagtatgcggagggaggtgggcccagccggctcacactgacggcaccctctccgccccagtctccag

SEQ ID NO: 11421 - RNA, 1277 nt, Homo sapiens
  source 1..1277: mol_type = other RNA
ctgaatagctgggactacaggtgcctaccactgcgcccggctaatttttgtatttttagtagagacagggtttcaccatcttggccaggctggtctcgaactcctgacctcgtgatccacctgtctcggcctcccaaagtgctgggattacaggcttgagccaccgcacccggccagaccctccagttttgtaaattgaaatggaaaaattaaattagtttgcaaatacaagatactgtctagcctacagatttcattacaaaattctgccttgtcataatccccaaaataattcagaacaaggcacaaaccagtgatttttttttttttttttgagacagagtctcgctctgttgcccaggctggagtgcagaggcacgatcttggctcactgcaagctctgcctcccgggttcatgccattctcccgcctcagcctcccgagtagctgggactacaggcgcctgccaccatgcccggctaattttttacattttttgtagagatggggtttcaccgtgttagccaggatggtctcgatctcctgacctcgtgatccacccacctcggcctcccaaagtgctgggattacaggcgttgagccactgtgcccggcctaaaatcagtgatttttaacttagcaaagtgggcttggcattttatccttatgtcaaaacacaagactaggctttcagtgaaatatcagatgagaattctccctctgcagcattatcacatgcgtcatcaattactgccatgcctaagtctagcatcatgccagcacattaagacagaaggtactatatgcagtgttcactggaccagaaagacagaaataagaaagggaggtggggagaaagaaaccctagagaagaaattaaaaaaaggcagaccgtgcaatacaaaccagatcatggctgcttagctaatatgggccaactgcgattctataggcttgtcaagtgacgcttgttcaatttccaagtgtccttcctcatactgatcaaagtgattaccctgaaagtctcggtcttcgttgaagcgggagaagcggtccgccattttgccgccttcactcctctcaggacgacgctctccggttcgctccttccctcctgcgacacccacccctccccggttccccgcctcctcccacgcccaccgggcgcgcgcagccgagggagggagcgagaatgcgcgtcctgacgggagccccgcggcgcaggcgcctgccagccctggaggctgacccttccctctagcccctgctccgcgcgc

SEQ ID NO: 11422 - RNA, 1303 nt, Homo sapiens
  source 1..1303: mol_type = other RNA
ctgaatagctgggactacaggtgcctgcaaccacgcctagctaattttttttttttttgtatttttagtagaggctgggtttcaccgtgttagccaggatggtctcgatcttctgacctcatgatctgcccacctcggcctcccaaagtgctgggattacaggcgtgagccaccacacccagccggtctcttggtttacaaatatagacaaatacataggaacactgactggtatttccatgtcaagaaacatggtcatatgtacagacaagacatggataaccaacaagttttaaagaaatgtatacatctctagttaaagattctaaccagaaatgctacgagagagctggcaaatgacaaccaccaatacatagatttctacactcctgaaaaagacaacaacatcaaaaaaaattaagaaatttggcatcaggtggacaacatctaggttttagggttaatatactgtttcatatactgtacaaagtttcatcattgcccccaaccttggaatttcagagtgagagcatatacaattcaaaacacttgctttgtcccttttctcagagctctgatattttcctaactcttacagtctctagaatgatctgtcagattttcactcaacaacactggatcagatctcttctatacatgacctcatccttctcatgtctcctctgtttgcagagagccggtcaaagtcttggaggtggaaacgaactgccaactgattaaccattttccttaaggtaagaaatgctgcaacaacttggaaagcaaggaagagagtgaagatgatatgtatcgctttttccaagggcagatttgttaggccttcattaaagagcaagaaaagaattaaaggtaactgcaatagaaggctcaaaagccaaaagccagccaactcaggaaccttctcctgtaggttacccacgtagcccagatacaaccggatggcttcaattaaggttattaggatgataacagtgatcacaatgaatttgtagtagtcaggtaagattgaatacttcatgtgaagcatcataatgctgctcacccaccacagtgggaaatagtaggtattaaaataaagtgacatctgcagtgccaaactggagaccatttcattttccggaccctcattggactctggaccggtccgattggaatcactgaacacggcccggctgaagtttcccagccgctggcgcaccggatccggcagctccatgcctgggcctcagtatccctcaccccctcagacacgggctagtctgcgggcgctccgaggctccgt

SEQ ID NO: 11423 - RNA, 1245 nt, Homo sapiens
  source 1..1245: mol_type = other RNA
ctgaatagctgggactacaggtgcctgcaaccacgcctagctaattttttttttttttgtatttttagtagaggctgggtttcaccgtgttagccaggatggtctcgatcttctgacctcatgatctgcccacctcggcctcccaaagtgctgggattacaggcgtgagccaccacacccagccggtctcttggtttacaaatatagacaaatacataggaacactgactggtatttccatgtcaagaaacatggtcatatgtacagacaagacatggataaccaacaagttttaaagaaatgtatacatctctagttaaagattctaaccagaaatgctacgagagagctggcaaatgacaaccaccaatacatagatttctacactcctgaaaaagacaacaacatcaaaaaaaattaagaaatttggcatcaggtggacaacatctaggttttagggttaatatactgtttcatatactgtacaaagtttcatcattgcccccaaccttggaatttcagagtgagagcatatacaattcaaaacacttgctttgtcccttttctcagagctctgatattttcctaactcttacagtctctagaatgatctgtcagattttcactcaacaacactggatcagatctcttctatacatgacctcatccttctcatgtctcctctgtttgcagagagccggtcaaagtcttggaggtggaaacgaactgccaactgattaaccattttccttaaggtaagaaatgctgcaacaacttggaaagcaaggaagagagtgaagatgatatgtatcgctttttccaagggcagatttgttaggccttcattaaagagcaagaaaagaattaaaggtaactgcaatagaaggctcaaaagccaaaagccagccaactcaggaaccttctcctgtaggttacccacgtagcccagatacaaccggatggcttcaattaaggttattaggatgataacagtgatcacaatgaatttgtagtagtcaggtaagattgaatacttcatgtgaagcatcataatgctgctcacccaccacagtgggaaatagtaggtattaaaataaagtgacatctgcagtgccaaactggagaccatttcattttctgctatatgaagcagctgctccatgcgtcaaccatgtgggagatgggaacgtcaagccgagggaagaaaatcagtaaagcaaaaacccgcttaaggaaacctcagat

SEQ ID NO: 11424 - RNA, 1321 nt, Homo sapiens
  source 1..1321: mol_type = other RNA
ctgaatagctgggactacaggtgcctgccaccaaccatgccctgctaatttttttgtgttttttgtagagacgggtgtctcaccatgttggccaggctagtcttgaactcctgacctcaagtgatccacctgcctcggcctcccaaagtcctgggattacagaagccaccgcgcctggccccaaggggaatcttttaaaaaagagaagttcccataaactgctttgaaaccataaagaccaaaggttagaagggtttgccgcaggcgctccgttgctaatgtttttgtgagggcttcttcagggcctcttgttagagtgtgacataaacgacttcatttgggtaccagcaagtgtcacagggggcagagaccagcagaaacctaaagatgacccctagaagagcaggaggccaggggaacagagttagacgagccacgtgctaagcaggacgtcgctgccgggggagctctccagacacgcagaaatgccacagtcaggaccgtgggacgcagcggattcgcccaagggcaggagcagcctggccaggagagaatgaaggaggggccgggcgtgaggttcggctggggagaacccaggcagggagggcctcgggcggccacggacgccgctttgccattttgggcgtttctggggaggacaacgcgtgcaggaagcgcagtcatctcaagctgacctccaaggttaccgagttcgagggctgggagccgggtctgaaagccccgacccgcctatggcgcggggactgtgggtccagccggccgattggccgcctcgctcggcgccggtccaggcgcagcgctcgggccccggggaccgtgagatgcggcgcagccagcttagctcggggtagcagccaccccagcccgggtgccgcccggcctggtccgcgacttcgggagggtccggtccttcccccggcccccacgcctgggtgaggccctgggcttcttgccggtgaccacgcggccagggtgggcaccagcccaggacggcgcccaagggcagcccagctccatccccgcgccgcgggttccggaaccgaggcgcgggacgctgggactctctgccaacatggcggccccgcccgggcgcctccccgggtccctagtgtctgcgtctcccgtgagggcgtgggcaaagtcggtgcagccagacgacaggaggcgagagaagcccagctccaggcccatgaggcgaaccacgtgggagccccagacagcgaccacgccccaggcgaaccaaggcccgccccgttgctacagctacgctcgtagcacacctgggcaggcgctgccggac

SEQ ID NO: 11425 - RNA, 1667 nt, Homo sapiens
  source 1..1667: mol_type = other RNA
ctgaatagctgggactacaggtgcctgccaccaagcccagctaatttttttgtattttttagtagaggcagggtttcaccatgttagccaggatagtctcaatctcctgacctcgtgatccgcctgcctcggcctcccaaagtagaactagctaaacttttattaacgtgctctacctagttcacattctcacaatttcaaattgaactacatcacatcctgagtagaaaatgaagatatgaacaatattgcagataaatattaaaactgaagatattaacacccttgccagttatttgttgacatttttcactcttgatattggtgtggtttattataacatttggcttagcacctaagtttgacaatgttttacaaaatccattcttaaatttctgcagtcctctatcatagcagatgactatctggtataagaaaagaaaagaaaagttggtcataaaataagttaaacactcctctcttttgtttgttcacttatgagttatatgtgaaacacatgagaaaaattcatgattttgacaatataaaggaaaatagattttaaaaaagaatgtaactgcctgtaaatataaataataattggtttcagtagacaaaaaataattcttaaatatgatgaataatccagttgtaaaatgtgtattattcctataagttggtttgaatacagacgtaaacatatatgtaaaatttagaagcaaagtagtaaacagaaaacgcaataagtagctgccgctaactcaataaattcttagagttggagattgaacttgcttttttgtccccaagatcacattcacttcatcttatgttcatgctttctcttttgccaggaaatatgttccaacagattttgccaacaatttcaatatttctgctgccatgtaagacatgcctttgctcctcctttgccttctcccatgattgtgaggtctccccagccatggggaaatgttgagtccattaaacctctttttctttataaactacccagtctcaggtatgtctttatcagcagcataagaacaaactaatacaaatgctgaggaagaatgatgtgattttttcactcatatagttcctcttccagtggtttggtgaagttgttagtagcaaaggcaggatgaagattttgtaaagagtggttcaaaaggcatagattaccctgaccaatacttctcaaaaactgaaaaggtcatcaaagccaaagaaagttctgaggaatagtggctgctaagatgagcttaaagagatgtgacaacttcatgtatgttgtatccttgatggtatctttgtgccatgtggagattaatccctttcttgaaggtgtcatgtagattgttgtttgtcagttgattgtgcaattgaacagtttaatcacttcttgctcttcattgcaggcaggaagagttggaaattagctttaagaagtctctttggcctctgtggttgctggcgtctcactcaggtttttgggtgccactgtgttcccctcatccagaccctggtacttgcagcggaagccgcctgtggtacacctggtccagctgcagcctcgcaaggagctggtgccggtgccggttcctggagctgcatgccctgccgcagcagctggcgtgcctggctgtgtgcagtggccagacccc

SEQ ID NO: 11426 - RNA, 5793 nt, Homo sapiens
  source 1..5793: mol_type = other RNA
ctgaatagctgggactacaggtgcctgccaccacacccagctaatgttttgtattttcagtagagacggggtttcactgtgttagccaggatggtcttgatctcctgacctcgtgatcttccccagggatggggtgttccatcttctgccctgtccggcagagtagctgcttgccacctgaggctgtcatgcacctgaaatgttggctagagggactgagaagctgaaatttcttatttctcattatttgaaattgcaggcacccatagcaagtggcatccatggtgcttggctttgaggtgccaggcaagcacagcttgttctggggcttggctgtaccagcagggggatgtgtttctggggaattgtggctctggaagcttcacggtttcccagaatgtggaaaatatatctgtgcaggatagaaatcctgcccagaggctgtttctgtctcatttgagctctccttcatgtggcagagctggctgtggcgtttaggagcctacattttagaaaagcttacctcaaagttctgcattgagcctgagactggaaaggagataaaataaaacagctgacaggagctttggtagtcacacatgcctgatggggtgcacagggccacagtctctgaaaggcaatttggcattgtctgtccacaatatacttttatccattggtccagcaatcctactctaggaatttttcctacatataaacctgtatgcatacaaaatgatagacatacaaggttattactctgaaaaagcaaaagattggaaacaaaccaagtgactggctacaggggactggtgaaatagagtatgttccatccacacagtggaattctgttcagcagtgaaaaaaggatgagagtgctttccaagtgttgttatggaaagagctccaggataaattaagtggaaaaaaaccccaagatacaggtacattaaaccgaaggaaattggttcagaggatagctgcaccatttttagagaaaaagcttcctttctctcttcaccttttgcaggtgatgtatttttttctttggattccttttttttttctttttttttgaaacagtttagcttggccgggcgcagtggctcatgcctgtaatcccagcactttgggagggcaaggcgggcagatcacgaggtcaggagatcgagaccatcctggctaacacagtgaaaccctgtctctactaaaaatacaaaaaattagccaggcatggtggcgggcacctgtagtcagtcgcagctacctgggaggctgaggtaggagaatggcatgaacccgggagacagagcttgcagtgagccgagactgtgccactgcactccagcctgggcgacagagcaagactctgtctcaaaacaaacaaacaaaaaaagagacagagtttcacgcttgttgccctgtctggaatgcagtggtgtgatcttggctcactgcaacctccgtctcttgggttcaagcaattctcctgcctcagtctccggagtagctgggattacaagcacacaccatcatgcccggctaatttttgtatttttagtagacaggtttcaccatgttggtgaggctggtcttgaactcctgacctaaggtgacccatccacctcagcctcccaaagtgctgggactacaggcatgagccacggagcccagccatttttggattcttaaaacttaagaaaaattctaaaacatatttgtgatctattacgttatgatatatgatagggaaaaaatagacaactttacctaccactaagttatatttaatcagcattcttttgtttcctaacatatatgttgcgagctaaatgtatgctcttactctaaatctttctgagctacactttaagggtgataattgttttgttttgttttttgagacagtcttgctctctcacccaggctggagtacaatggcgagatctcagctcacggcaacctccgcctcccgggttcaaatgattcttgtgcctcagcctcccgagtagctgggattacaggtgcatgccatcacagctggctaatttttgtatttttagtagagatggggtttggccatgatggccaggctggaaaattgaaacataatttcacaattattcctttttccaccttaaataataagagtagaatactttctgtgtttttatcttatacacatgaataaatgctatggcttatcacagttacaatgtgttttctgaaagtaaagattattttaccttgaaattacaaaaattattttcagttttccaaaattctatctttaaacctaaataattcaatttcatggatgcacaaatgtttattgagagtctcatattcatgcttttcttcacagcactataaagttggacttggaaaatttggacagccatttgccattgtaatttttattcttttttctcctgattatttgacaaaacttgtatccacattgtagctgttcatgtgtctgcttctattgcatattgtaaaattattaactacttcccaaaatagtatttctctcagcagatatttctttggtactaccatgtattgtgtaacttttgggaaagtaaggtggcttccctgctctcagtgaagcattttattaaaagaataattataattaaaaaaacacgatacagatcagtgcatatagtatattactaatagtatgctgttaattgtgtaagaaagaaaggaaattagaaaacatatttgcataaataaaagctagacaaaggctaagaaactaatcaggtggtttccctggggtagtaggataatggggaacagtggggctgggaccgggtgggagaaagagttctcagtggttcctttctatacagttttaacttttgaaatgtgtgagagtgttacttactgaaaactgaaaggatatgacatgctggaacaggcaaaactacaaagacagtaaaaagatcagtgatttccaggagctgcaagggcagtgagaggaagggagggatgaggaggtggagcgcaggggatgttagggcagtgaaaggttctgtatgacactgtgatggtgggtacatgacattgggcattggtcaaaacccatagcatgtacagcacaaagcgtttgctctaatgtgagctatggactttagttaatagtaacgtgtcaatattggttcatcagttgtatcaaatgtaccacactgatgccagatgttaataatcggggaaactgtgtgtgctgaagagtacgtgggagctctctgtgctatctgctcaatttttctctaaacctaaaactgttctaaaatagaaagtctgtgaaaaaaaacaaaagtaaagttataaaaggaaaagaaaacagaggctttaaattaaatcatctattccttgggaaaggtattttgtaccatatgggactgaaatcatttatctggatgaattttataaaatgaattttgtaatttttttctgagaaaaaaaagttcttaaatacaataaaattgaaatgttgaaatatatctctcaaatccagtactcatatcttttctttgggaaatacagggtgaaattccaggtcagacaagctgtcacagattggtgctatgtaagcacaatggctcaactcacggacagtgaatacttcctgagtggattttgtgccaggtggcctgccaggagtgggtacagagatgagagcccacagttccctccccttccccaagcttagggtctagtaggggagaaaggcttgcacaccaataactgtaataaggtgcagtccacgctgtaatggatgggtgcaaacaactatgggactccttcctgggggaaggaagaaaggaaggggaggaagcagctcacagaggagacagaagtggggaaaagggcagtccaagccaacagcacagcctaagcaatagcccagaggtgtggagagggaccccccaccttggggagtagcgtggctggagcacaggatgcgtggaaggagggggagctgtgacctgaggggcaggagggggaggggtgcagatgcattggaaattgttccccaccccatcaccaaaaattagatgtctcataaagtagaaactgaacagaatagactccgcctttggaaatgcacatctgcttgtcctttcagagtctactttaccttgctaattgtgactctccttgtttctaaaatgtatatttaaatcacttttccaatggatatttacttacagttactccctcccttttctttgagacggagtcttcctctgttgccaggctggcgtgcagtggtgcgatctcggcttactgcagcctccgactccctggttcaagcgattctcctcttcagcctcccaagtagatggaattacaggcacatgccaccacgcccagctaatttttttttgtatttttagtagcgatggggtttcaacatgttggccaggatggtcttgatctcctgacctcgtgatctgcctgggttggccttccaaagtgctgggattgcaggcgtgagccactgtgcctggcccctttttaagatatatactgtacttaaaactattcacatatagtctgcaggtttatatacttaaaaagtgcgaagtctttctcctgtggatcccaagataacttctagaagcgggtacaggccctggatcacatcatgtatcaaaatgaacccataaaactcccaggttaagaactgaggtgaaggagtccctggctcttagtggaggttgctccccgcatctcttcctgtgtgcagagcttcactaaatggttacagccccacttcagagtttctgaaactagtctgatttccacaacagaggtcccttagtgttcatgcactggcaagtgacaagatcagacctgtgtgtggaccacacagaggatgggtgggggtgggaggagatggctggtggagccagtgaggactgtagtagtctgggcaaaagatgccaaggcctaacttgtagtgaggaaggctcaagtttgcaggcaagttgctagatctctgagagtcaggggatataggtgtagtagatgtggaaatgcattgcccggacccccttcttccaggaaggcctttccatccagctgcaggagtgagctgggcagatggcctccagctgtcagcccttcagggtctgcctcagctgcagagagttgccccacccaacaccctgccctccccagggcagctgcctctgggaactgagctacgcgggagcatagagacccagccattttagtcctccatgaaaatattccagtgggtgcttcaagctcctgcgtgccctactgagttggtgggtacttgatcgggcctgcatcacagttcaatttcgctctctgcccaatccatcttcccttcacagatgttgtttttttgttttgttttggagattgagtctcactctgttgctcaggctggagtgcagtgacaccatctcagctcaccgtaacctctgccactctggttcaagtgattgtcctgcttcagcctcctgagtagctgggattacaggcacgtgccgccaggtctggctaatttttttgtatttttagtagagactgggtttctccatgttggcctggctggtcttgaactcctgacctcaggtgatccactccccttggcctcccaaagtactgggattacaggtgtgagccaccacaccaggccacagatgttgatccttaataaacatcttgcacccaaattttcatctctgcatccgcttcagcctgtaatctcagctacttgggaggctgaggcagaagaattgc

SEQ ID NO: 11427 - RNA, 2396 nt, Homo sapiens
  source 1..2396: mol_type = other RNA
ctgaatagctgggactacaggtgcctgccaccacacccagctaattttttttttttttttttttttgtatttttagtagagatggggtttcaccgtgttagccaggatggtctcaatctcctgacctcatgatccacctgcctcggactcccaaagtgctgggattacagacgtgagccactgcgccctgccagcttcactaaatttttaaggcttctctctggtatgaatactgcaatgttgtactaggatggaatttttactaaagaccttgccacattcattacaactgtaaggcttcactccagtatgaatattcctatgttgtgcaaggcgtgaattccgactgaagaccttgctacattcattacatttgtaaagcttctctccagtatgaattttcctatgtcgcgcaaggtgtgaattccgactgaagaccttgccacattcattacaactgtgaggcttctctccagtatgaatattcctatgtcgcgcaaggtgtgaattccgactgaagaccttgccacattcattacaactgtaaggcttttctccagtatgaacattcctatgtcgcacaaggtgtgaattccgacggaagaccttgccacattcattacaactgtaaggcttctctccagtatgaatatccctatgttgtgcaaggtgtgaattctgacggaagaccttgccacattcattacatttgtaaagcttctctccagtatgaattttcctatgtcgttgaaggtttgaattctgactgaagaccttgccacattcgttacatttgtaaggcttctctccagtatgaattctacagtgataggttagggaagacttgtgcctgaagaccttgccacagtctatacattcgtaaggtttctctccagtatggattagaagatgggcagtgagatctgaacacgttctaaatgctttgccacattcattacatttgtaacgcctccccccagtatgaattttcctatgtcgtgcaaggcgtgaattgccaataaagaccttgccacactcattacatttgtaaggtttctctccagtatgaactttccgatgccttgcaaggaatgcaattcgactaaaccccttgccacattcattacatttgtatggtctctctccagtatgaactgtctgatgagtggttagggaagacttatgcctgaagaccttgccacattccttacaatcataaggtttctctccagtatggattacaagatgagcagtaagactggaacacacactaaatgctttgccacattcactacatttgtaaggcttctctccagtatgaattttcctatgctgtgcaaggtaggcatggtgactaaagactttcccacattctttgttattgtaaggtttctgtccagtatgaattttctgatgttgtgcaaggtgtgaattctgattgaagactttgccacattcattatatttgtaaggcttctctccagtatggattcgttgatgttgtgcaaagtttgaattgctactaaagatctcgccacagtcactacatttgtaagttttatctgcaatgtggattacttgacggttagtaaggcttgaagacactctgaagactttcccatgctcattacatccataaggcttttccctaatgtgtactttctgttcttgtgggagtaatgtagaaaaaagaaaatcatttctgtagttattaaaaatatgggttttgacactgaaaaaacttatttgaactggtgaaactgaagaattgtcactgatagatttctcaacatgcttacatccataaatattccttacagcttgaaatggctgccattcagtcagatgtaactgaagagttaatccatgttgatttttaagtgacttgtttcctgcactgcttcccaatttagaactcttctctgtgttcacacctttgatgcactccctgccatctggattgtttattattttcacttcactctgcagagtccagggatctctcttttgctccaacatggaggtaacactcaggtcaggaagacagattccagagcagatgcaggcttctggacggacattatcctcacctagggagaccaggttcctgtagttctctaacatcacgtccctgtataaagctttctgcccagggtccaggcatttccactcctcctgagagaattctatggccacatcgctgaatgacaattgcccctgagtaagggccattcctgacttcctttctttcctcttccgagttgcttccttgcataatatgtctctttgaaagtgaatcgagtggcggcttagacagtctttccgcgcagtcgggtgccgggtctacaggaaaaagcgcgcgaaacgttcactccatgatctcgacttccgggtct

SEQ ID NO: 11428 - RNA, 2357 nt, Homo sapiens
  source 1..2357: mol_type = other RNA
ctgaatagctgggactacaggtgcctgccaccacacccagctaattttttttttttttttttttttgtatttttagtagagatggggtttcaccgtgttagccaggatggtctcaatctcctgacctcatgatccacctgcctcggactcccaaagtgctgggattacagacgtgagccactgcgccctgccagcttcactaaatttttaaggcttctctctggtatgaatactgcaatgttgtactaggatggaatttttactaaagaccttgccacattcattacaactgtaaggcttcactccagtatgaatattcctatgttgtgcaaggcgtgaattccgactgaagaccttgctacattcattacatttgtaaagcttctctccagtatgaattttcctatgtcgcgcaaggtgtgaattccgactgaagaccttgccacattcattacaactgtgaggcttctctccagtatgaatattcctatgtcgcgcaaggtgtgaattccgactgaagaccttgccacattcattacaactgtaaggcttttctccagtatgaacattcctatgtcgcacaaggtgtgaattccgacggaagaccttgccacattcattacaactgtaaggcttctctccagtatgaatatccctatgttgtgcaaggtgtgaattctgacggaagaccttgccacattcattacatttgtaaagcttctctccagtatgaattttcctatgtcgttgaaggtttgaattctgactgaagaccttgccacattcgttacatttgtaaggcttctctccagtatgaattctacagtgataggttagggaagacttgtgcctgaagaccttgccacagtctatacattcgtaaggtttctctccagtatggattagaagatgggcagtgagatctgaacacgttctaaatgctttgccacattcattacatttgtaacgcctccccccagtatgaattttcctatgtcgtgcaaggcgtgaattgccaataaagaccttgccacactcattacatttgtaaggtttctctccagtatgaactttccgatgccttgcaaggaatgcaattcgactaaaccccttgccacattcattacatttgtatggtctctctccagtatgaactgtctgatgagtggttagggaagacttatgcctgaagaccttgccacattccttacaatcataaggtttctctccagtatggattacaagatgagcagtaagactggaacacacactaaatgctttgccacattcactacatttgtaaggcttctctccagtatgaattttcctatgctgtgcaaggtaggcatggtgactaaagactttcccacattctttgttattgtaaggtttctgtccagtatgaattttctgatgttgtgcaaggtgtgaattctgattgaagactttgccacattcattatatttgtaaggcttctctccagtatggattcgttgatgttgtgcaaagtttgaattgctactaaagatctcgccacagtcactacatttgtaagttttatctgcaatgtggattacttgacggttagtaaggcttgaagacactctgaagactttcccatgctcattacatccataaggcttttccctaatgtgtactttctgttcttgtgggagtaatgtagaaaaaagaaaatcatttctgtagttattaaaaatatgggttttgacactgaaaaaacttatttgaactggtgaaactgaagaattgtcactgatagatttctcaacatgcttacatccataaatattccttacagcttgaaatggctgccattcagtcagatgtaactgaagagttaatccatgttgatttttaagtgacttgtttcctgcactgcttcccaatttagaactcttctctgtgttcacacctttgatgcactccctgccatctggattgtttattattttcacttcactctgcagagtccagggatctctcttttgctccaacatggaggtaacactcaggtcaggaagacagattcctagggagaccaggttcctgtagttctctaacatcacgtccctgtataaagctttctgcccagggtccaggcatttccactcctcctgagagaattctatggccacatcgctgaatgacaattgcccctgagtaagggccattcctgacttcctttctttcctcttccgagttgcttccttgcataatatgtctctttgaaagtgaatcgagtggcggcttagacagtctttccgcgcagtcgggtgccgggtctacaggaaaaagcgcgcgaaacgttcactccatgatctcgacttccgggtct

SEQ ID NO: 11429 - RNA, 2230 nt, Homo sapiens
  source 1..2230: mol_type = other RNA
ctgaatagctgggactacaggtgcctgccaccacacccagctaattttttttttttttttttttttgtatttttagtagagatggggtttcaccgtgttagccaggatggtctcaatctcctgacctcatgatccacctgcctcggactcccaaagtgctgggattacagacgtgagccactgcgccctgccagcttcactaaatttttaaggcttctctctggtatgaatactgcaatgttgtactaggatggaatttttactaaagaccttgccacattcattacaactgtaaggcttcactccagtatgaatattcctatgttgtgcaaggcgtgaattccgactgaagaccttgctacattcattacatttgtaaagcttctctccagtatgaattttcctatgtcgcgcaaggtgtgaattccgactgaagaccttgccacattcattacaactgtgaggcttctctccagtatgaatattcctatgtcgcgcaaggtgtgaattccgactgaagaccttgccacattcattacaactgtaaggcttttctccagtatgaacattcctatgtcgcacaaggtgtgaattccgacggaagaccttgccacattcattacaactgtaaggcttctctccagtatgaatatccctatgttgtgcaaggtgtgaattctgacggaagaccttgccacattcattacatttgtaaagcttctctccagtatgaattttcctatgtcgttgaaggtttgaattctgactgaagaccttgccacattcgttacatttgtaaggcttctctccagtatgaattctacagtgataggttagggaagacttgtgcctgaagaccttgccacagtctatacattcgtaaggtttctctccagtatggattagaagatgggcagtgagatctgaacacgttctaaatgctttgccacattcattacatttgtaacgcctccccccagtatgaattttcctatgtcgtgcaaggcgtgaattgccaataaagaccttgccacactcattacatttgtaaggtttctctccagtatgaactttccgatgccttgcaaggaatgcaattcgactaaaccccttgccacattcattacatttgtatggtctctctccagtatgaactgtctgatgagtggttagggaagacttatgcctgaagaccttgccacattccttacaatcataaggtttctctccagtatggattacaagatgagcagtaagactggaacacacactaaatgctttgccacattcactacatttgtaaggcttctctccagtatgaattttcctatgctgtgcaaggtaggcatggtgactaaagactttcccacattctttgttattgtaaggtttctgtccagtatgaattttctgatgttgtgcaaggtgtgaattctgattgaagactttgccacattcattatatttgtaaggcttctctccagtatggattcgttgatgttgtgcaaagtttgaattgctactaaagatctcgccacagtcactacatttgtaagttttatctgcaatgtggattacttgacggttagtaaggcttgaagacactctgaagactttcccatgctcattacatccataaggcttttccctaatgtgtactttctgttcttgtgggagtaatgtagaaaaaagaaaatcatttctgtagttattaaaaatatgggttttgacactgaaaaaacttatttgaactggtgaaactgaagaattgtcactgatagatttctcaacatgcttacatccataaatattccttacagcttgaaatggctgccattcagtcagatgtaactgaagagttaatccatgttgatttttaagtgacttgtttcctgcactgcttcccaatttagaactcttctctgtgttcacacctttgatgcactccctgccatctggattgtttattattttcacttcactctgcagagtccagggatctctcttttgctccaacatggaggtaacactcaggtcaggaagacagattcctgagtaagggccattcctgacttcctttctttcctcttccgagttgcttccttgcataatatgtctctttgaaagtgaatcgagtggcggcttagacagtctttccgcgcagtcgggtgccgggtctacaggaaaaagcgcgcgaaacgttcactccatgatctcgacttccgggtct

SEQ ID NO: 11430 - RNA, 4550 nt, Homo sapiens
  source 1..4550: mol_type = other RNA
ctgaatagctgggactacaggtgcctgccaccacacccggctaattttttgtagttttagtagagatggggtttcaccgtgttagccaggatggtctcgatctcctgacttcatgatctgcccgcctcggcctcccaaagtgctgggattacaggcatgagccaccgtgcccggccgcgagaataaactttcaaagtacccatttgtagagattttttaattgataaaattcactgagtagtgggcccttctgatgggcaggactttcagatcattcagatgacataattagtttcttaggagttctctatgctctacttgcaattctcataaattctgtttcacctctcaatttatactcatagatgtacactctaaaatgtggtcctgtggctggatggggtagcgcccaagtggaaaagcatatgggtgaaggtgctgccctgagtagccctttagcctttttagatgaaacttgaacttacagtagaacatttcccatacagagacccaaattaaattctataactctttacttcacaactagtggttggaggaggtggcatattggctcttctcacataaatatctataacagcggtgcctgtcctgggcttggtggatttgccatatttcaagttatcatcaattatatgcacaacaagatggtactgctgctgtacttcagctctacattcaaagttgaaaggattcttcacaattaattttggagtatttgaacctcgagttgggtcaaatccaaaatgatggttctcttttcctttaaaagtgataattgagaagttagaattattttaaggtatattgaaagattttctcaaactaccttaaattgctattaaaacacagtaggcgtaaatttttttaaaatttccattgcaccctgagtttttatatctatacatggcttataataaagctgagatcaaatgagcaacaatttcagttggttaggaaaaaaaaattttgaagattaagatcatgaatctgatcccatatatagccagcaagcctcaaattattatctaattgattctcctttccttctactcagatcaatttgattcccatcttcaacttagtctagatcaatatcaaatgggccggtcagatcataaatatctattgagccccttctaattttaagttatctccatagccctggagacattgttgatacacagggtccctaccttcatggagcttatcacccagcaagggaataagacatcaaactagtctttataatcaattggcaatgtccttactgatttccaagcttctactccttcagatacatgacagcaggtctgatctccataatttaaataggtctccacgttatgctgtctcatgatacccagtagttttcttttatagaacttatcacagtatgtaattttataattgctggtgttactactagtttagtaaacaatgagtgccgtgaatatctgtctcatatacttctgtgtacacatttccgagcacattgcctgatacatagttggtcccaatatatgcctttcgtaaaaaataagatggcttaagttgatatggatctgtgcaaatccaaaaataacacagtttgaaaccacgcatcctactgaatctgtactaatagcatcaaatggaaaggtggctgttgttatccagtaccatggacagcagacttcattccttgtaacttaaccttcaacatttcccatccaggttcaaagtccgttgtcaaagcatctgtaaaattactgatacttccattatgggaggaattagatttgatatgtgaaagtaaaaaagatgccttgaggaaacaatgctatagatattaaatagtttaactgttataaacataattatttctgaagttatacataatatctaacagggcaaaactaatgtcaatttgacatatgctcacgattaaaagaaataataaaattatgcaccagaaaccatctcaaaacgcatttcaaaatcttgtgactctccgtcgtggcagttcagggtgaagccattgacatttgtcccaagaacaacattgtcaaaaatgactgtcttatatagagagggtgtgcagacaggtgcttcatcattctcattttcaatgtcaacagtgatctgtcagccatgagggaagaagaaacatcaaatccacaccatgtgactacttatacacaatatcagaaataagcataagggtagagacggatcatttggaattattaaataaaaagtctagagatttggatttaaaaaaaatgttcctgcagattggaattctggccatcaatcaactagtcagtggtttattattcctgggttaactgtgacattcaatgtagccgttaggtaggattttggctcattagataagcttgtggaaagctcacaaattatgtaaatgatgagaaaaggaaagctgaagaatgatgcctctagaaattgtaatcccttgaactctttaaatatctatgcttaaaggcatagataaatttgcttcctctttctcaaaagaacttcctcagtactactctctcaaactcaatattttattggtaacaatatgattacttcaaagtatgctctgaccttaattagggactgttatcaaccttttcttaattaaaataccataaactaggaaactataatttacgtagaaaaagatcaaaatatcaagaatttttaaatgtcagtgattgaataccagtcagcctagaaaggttatctacccacttcttagatgactaataactgtctcaataatacttgcagaagaatccgtggtgcaccaatatttgcaagtattatctttttaaagtgttttatgtaatgttttaaaaacatagctaaattcttaaggaatggttcattctttaatgctacttctatagactgaatacagctatgtgtctcaccaagtatgtgagactttttacataataattaaacggattttaaggagatttctggaatagtccagtgctatttccattatatcacagaaagatatcaggaatctttattaaaatcctgggcctgacacttattgatgactttatttggcactagtgacttaccttttctttcttcaactgcaaaaagcagatctcaatctctaccttctcaggactgtcagaaggatcagttcattcattcagtgaatatttattgaatacttactatgtgccaagcactgatctagacaccacagaagctacagtggtaaaccaaaaacaaagaccctgatctaatataatttattctaatgacgaaagcaaagcaataactatactgacaaataaatatattaggcaaaatcataggataagctgatgctatttgggttaaggagatagagaatagctgatggaagtattttaagagggatttatttctttgacccactcacctattccctctctctcatgtttgttatatgtccttaagcatgtatgtatcctcatagaatatgtagcttttagttgtataattttgacttgcacaaatgatatggtgctatagaccttttgtgtttcttacttttctcacccagcgccatatatgtgctttccatgtttttgtttgcagaattcatttgctatttctggagtctgtattctgtagtatgcatctaccatatttgcttgttcatttcccatgatgaacacacatggattgcttcaaatgcccaccattacacacaatataaaaggcccttagaaacaaatttcatttgggcagagatatgattaaagtgagaatatgagccaatggaagataagcattacagtctttggcagaggttctgaggtaaaacattgttggtgtgttggaaaaacaacaaatgtttcatgtggctggattgaagtaagtaagagggagagagctaggagctaaagacaaattggtagccagggcccagatcatagagggcactgcagactttgaagatgacattggagcttaactaagcatgatgggaagccaatggagaatgttgaggaacaggatgatttatctttttaaaaggtcactctggctgtggtgtgaagagtaggctgtgaagggcacaagtaggaatgggggttctaatcaagaagctgctacactagaccaggtgaggtatggtaaaggcacagttggggtattagcagtagacaagttagaaaagtaagaagtggaaggacttaaggtacattctgaaattagagaagacagaaattgctgttggattggagaaataatttagggtacatgatagtgattaagtactcagacttaatccttctccttctttcagatgggtaatcttggataagctacctaactttgaagccttggaaataaaattcttccatctgttaaaaggagtatcagtaactattccataagatgagattaaattctaaatgagataatcaagggcatttcatagcacttgacttttattagattctcaataatgagtgggtgatgatgatagtgatgatgatgatgatgatagtgatgatgatgatgatgat

SEQ ID NO: 11431 - RNA, 1155 nt, Homo sapiens
  source 1..1155: mol_type = other RNA
ctgaatagctgggactacaggtgcctgccaccacacccgggtgatttttgtatttttagtagagacggggtttcgccatgttgctcaggctggtctcgaactcccgacctcaagtgacttgctcaccttggcctcccaaagtgctgggattacaggtgtgagccactgcacccagcctggcagtcaattttaagcctcctatttcccaggttttagcttaataatcctcattagtttttcagatttttgtcagtcttgttttggggctattttgccttagtgggcctaaacagaatattaaaatacattaataatccatactgagagtagagtataaatgggtttctcactccttagggacacgagtggaaacaatacatcccatgaacacaggtgaatgtccctggttatccctgagctgggcagtttcacacaatcattttttctctgaggccaaagtctgtggtttgatcatcttagcagcttccagaacagaaagtaggtttactttgtctccaaattctttttctcggtgctcaagaagaatgccctgctttcctgatcccaccacgaaaactcccccaaggatgaagccttctccttccaggtttccagagaagcctccgttccaggctcggaagaagttgtaccacactcccagacggataaatcccataaacatcatcttccgcctttgtggaccatagaactttttcttttcatccaggaagatttctcctttgaaataaggctggaaatccttcacttcagtcctgatgtgctcctttaccactgcatagagggggacgcccagctggtccaacatgcttttcagggaggacagatccgcagcttcctctcgacagaggaaacagcctggcctccgcacggccataatcacagctccatttttttcccatagctcctttgctttgaaagtccttggttccttctccagtgttttcaggtctatatcctccaggtactccagggccgctttctggggcttggacagaaacacgtctgtgttggcaagcagcaatgccaaggcagcagcccccagggctcctgcaccaatggaccacatccccatggtgaagaaacttgggtccatacacagcgtccacacctctgcttctcttgacaaagaagtat

SEQ ID NO: 11432 - RNA, 1204 nt, Homo sapiens
  source 1..1204: mol_type = other RNA
ctgaatagctgggactacaggtgcctgccaccacacccgggtgatttttgtatttttagtagagacggggtttcgccatgttgctcaggctggtctcgaactcccgacctcaagtgacttgctcaccttggcctcccaaagtgctgggattacaggtgtgagccactgcacccagcctggcagtcaattttaagcctcctatttcccaggttttagcttaataatcctcattagtttttcagatttttgtcagtcttgttttggggctattttgccttagtgggcctaaacagaatattaaaatacattaataatccatactgagagtagagtataaatgggtttctcactccttagggacacgagtggaaacaatacatcccatgaacacaggtgaatgtccctggttatccctgagctgggcagtttcacacaatcattttttctctgaggccaaagtctgtggtttgatcatcttagcagcttccagaacagaaagtaggtttactttgtctccaaattctttttctcggtgctcaagaagaatgccctgctttcctgatcccaccacgaaaactcccccaaggatgaagccttctccttccaggtttccagagaagcctccgttccaggctcggaagaagttgtaccacactcccagacggataaatcccataaacatcatcttccgcctttgtggaccatagaactttttcttttcatccaggaagatttctcctttgaaataaggctggaaatccttcacttcagtcctgatgtgctcctttaccactgcatagagggggacgcccagctggtccaacatgcttttcagggaggacagatccgcagcttcctctcgacagaggaaacagcctggcctccgcacggccataatcacagctccatttttttcccatagctcctttgctttgaaagtccttggttccttctccagtgttttcaggtctatatcctccaggtactccagggccgctttctggggcttggacagaaacacgtctgtgttggcaagcagcaatgccaaggcagcagcccccagggctcctgcaccaatggaccacatccccatggtgaagaaacttgggtcctcaagtgcctcccttctgccggccttttaccgccccgacgcccgggcgctaaggggccaaaccgcccggcccggagggtcccaggggcgggc

SEQ ID NO: 11433 - RNA, 1172 nt, Homo sapiens
  source 1..1172: mol_type = other RNA
ctgaatagctgggactacaggtgcctgccaccacacccgggtgatttttgtatttttagtagagacggggtttcgccatgttgctcaggctggtctcgaactcccgacctcaagtgacttgctcaccttggcctcccaaagtgctgggattacaggtgtgagccactgcacccagcctggcagtcaattttaagcctcctatttcccaggttttagcttaataatcctcattagtttttcagatttttgtcagtcttgttttggggctattttgccttagtgggcctaaacagaatattaaaatacattaataatccatactgagagtagagtataaatgggtttctcactccttagggacacgagtggaaacaatacatcccatgaacacaggtgaatgtccctggttatccctgagctgggcagtttcacacaatcattttttctctgaggccaaagtctgtggtttgatcatcttagcagcttccagaacagaaagtaggtttactttgtctccaaattctttttctcggtgctcaagaagaatgccctgctttcctgatcccaccacgaaaactcccccaaggatgaagccttctccttccaggtttccagagaagcctccgttccaggctcggaagaagttgtaccacactcccagacggataaatcccataaacatcatcttccgcctttgtggaccatagaactttttcttttcatccaggaagatttctcctttgaaataaggctggaaatccttcacttcagtcctgatgtgctcctttaccactgcatagagggggacgcccagctggtccaacatgcttttcagggaggacagatccgcagcttcctctcgacagaggaaacagcctggcctccgcacggccataatcacagctccatttttttcccatagctcctttgctttgaaagtccttggttccttctccagtgttttcaggtctatatcctccaggtactccagggccgctttctggggcttggacagaaacacgtctgtgttggcaagcagcaatgccaaggcagcagcccccagggctcctgcaccaatggaccacatccccatggtgaagaaacttgggtcctggaggaaagacatttcatacacagcgtccacacctctgcttctcttgacaaagaagtat

SEQ ID NO: 11434 - RNA, 1221 nt, Homo sapiens
  source 1..1221: mol_type = other RNA
ctgaatagctgggactacaggtgcctgccaccacacccgggtgatttttgtatttttagtagagacggggtttcgccatgttgctcaggctggtctcgaactcccgacctcaagtgacttgctcaccttggcctcccaaagtgctgggattacaggtgtgagccactgcacccagcctggcagtcaattttaagcctcctatttcccaggttttagcttaataatcctcattagtttttcagatttttgtcagtcttgttttggggctattttgccttagtgggcctaaacagaatattaaaatacattaataatccatactgagagtagagtataaatgggtttctcactccttagggacacgagtggaaacaatacatcccatgaacacaggtgaatgtccctggttatccctgagctgggcagtttcacacaatcattttttctctgaggccaaagtctgtggtttgatcatcttagcagcttccagaacagaaagtaggtttactttgtctccaaattctttttctcggtgctcaagaagaatgccctgctttcctgatcccaccacgaaaactcccccaaggatgaagccttctccttccaggtttccagagaagcctccgttccaggctcggaagaagttgtaccacactcccagacggataaatcccataaacatcatcttccgcctttgtggaccatagaactttttcttttcatccaggaagatttctcctttgaaataaggctggaaatccttcacttcagtcctgatgtgctcctttaccactgcatagagggggacgcccagctggtccaacatgcttttcagggaggacagatccgcagcttcctctcgacagaggaaacagcctggcctccgcacggccataatcacagctccatttttttcccatagctcctttgctttgaaagtccttggttccttctccagtgttttcaggtctatatcctccaggtactccagggccgctttctggggcttggacagaaacacgtctgtgttggcaagcagcaatgccaaggcagcagcccccagggctcctgcaccaatggaccacatccccatggtgaagaaacttgggtcctggaggaaagacatttctcaagtgcctcccttctgccggccttttaccgccccgacgcccgggcgctaaggggccaaaccgcccggcccggagggtcccaggggcgggc

SEQ ID NO: 11435 - RNA, 1589 nt, Homo sapiens
  source 1..1589: mol_type = other RNA
ctgaatagctgggactacaggtgcctgccaccacacccgggtgatttttgtatttttagtagagacggggtttcgccatgttgctcaggctggtctcgaactcccgacctcaagtgacttgctcaccttggcctcccaaagtgctgggattacaggtgtgagccactgcacccagcctggcagtcaattttaagcctcctatttcccaggttttagcttaataatcctcattagtttttcagatttttgtcagtcttgttttggggctattttgccttagtgggcctaaacagaatattaaaatacattaataatccatactgagagtagagtataaatgggtttctcactccttagggacacgagtggaaacaatacatcccatgaacacaggtgaatgtccctggttatccctgagctgggcagtttcacacaatcattttttctctgaggccaaagtctgtggtttgatcatcttagcagcttccagaacagaaagtaggtttactttgtctccaaattctttttctcggtgctcaagaagaatgccctgctttcctgatcccaccacgaaaactcccccaaggatgaagccttctccttccaggtttccagagaagcctccgttccaggctcggaagaagttgtaccacactcccagacggataaatcccataaacatcatcttccgcctttgtggaccatagaactttttcttttcatccaggaagatttctcctttgaaataaggctggaaatccttcacttcagtcctgatgtgctcctttaccactgcatagagggggacgcccagctggtccaacatgcttttcagggaggacagatccgcagcttcctctcgacagaggaaacagcctggcctccgcacggccataatcacagctccatttttttcccatagctcctttgctttgaaagtccttggttccttctccagtgttttcaggtctatatcctccaggtactccagggccgctttctggggcttggacagaaacacgtctgtgttggcaagcagcaatgccaaggcagcagcccccagggctcctgcaccaatggaccacatccccatggtgaagaaacttgggtcctggaggaaagacatttctgcctcagtctccaactctcagccctgctccttggggtgtgtatctgcctggttctggcccagtcctactctcaaatgccagattcagaaacctctgaatagatgctgaaagcagcaccagcccccacattcctcactcttgggcgtatctcagggtttcccagtagctgattatgtcctcttgtttcctcaagctgtagggccccccacccctcaaagagcaagccattctaatctcacttgcacagcctcctgtctgggctcagaactccggcttcatcaagttatatgggtgtggataggaaggcaaggcaataccacagaagacactgggctaaaagccaataatcctgggttttctctctttgactctgagagttattttatccctctgaacctcagtgtcttcttaaaaacaagggcactttaaagagttgtcataaagattatataagaagag

SEQ ID NO: 11436 - RNA, 1687 nt, Homo sapiens
  source 1..1687: mol_type = other RNA
ctgaatagctgggactacaggtgcctgccaccacacccgggtgatttttgtatttttagtagagacggggtttcgccatgttgctcaggctggtctcgaactcccgacctcaagtgacttgctcaccttggcctcccaaagtgctgggattacaggtgtgagccactgcacccagcctggcagtcaattttaagcctcctatttcccaggttttagcttaataatcctcattagtttttcagatttttgtcagtcttgttttggggctattttgccttagtgggcctaaacagaatattaaaatacattaataatccatactgagagtagagtataaatgggtttctcactccttagggacacgagtggaaacaatacatcccatgaacacaggtgaatgtccctggttatccctgagctgggcagtttcacacaatcattttttctctgaggccaaagtctgtggtttgatcatcttagcagcttccagaacagaaagtaggtttactttgtctccaaattctttttctcggtgctcaagaagaatgccctgctttcctgatcccaccacgaaaactcccccaaggatgaagccttctccttccaggtttccagagaagcctccgttccaggctcggaagaagttgtaccacactcccagacggataaatcccataaacatcatcttccgcctttgtggaccatagaactttttcttttcatccaggaagatttctcctttgaaataaggctggaaatccttcacttcagtcctgatgtgctcctttaccactgcatagagggggacgcccagctggtccaacatgcttttcagggaggacagatccgcagcttcctctcgacagaggaaacagcctggcctccgcacggccataatcacagctccatttttttcccatagctcctttgctttgaaagtccttggttccttctccagtgttttcaggtctatatcctccaggtactccagggccgctttctggggcttggacagaaacacgtctgtgttggcaagcagcaatgccaaggcagcagcccccagggctcctgcaccaatggaccacatccccatggtgaagaaacttgggtcctggaggaaagacatttctggagattgagaagaaggaagaaggcgttactgctcccacagggtagctggaatttcatcttccaggcaaggctctggcaggacagccaaccaggaggtcaggacaggggaagggagcagcagtgtcacaggcgagactggacaagggctgctaagcacctgctgccaccagaacttggggatgcagcacacacatggaggttcctgcaccgtggagctcaccagggcatcaggagtgatgacagagaaaggacagccttctcaaatggttctcttgctgctctctcttctcatgccccaagttgcagcccctagctctgtggagctgtgccgagctatgtcccctgtaggcagactacttcctcattcccctcctcatcaatgcctgattctccctcacaatccaggtggctcaggatcatgtccctgggtaggggcagctttctcttctgtgatcagaggatactcaagtgcctcccttctgccggccttttaccgccccgacgcccgggcgctaaggggccaaaccgcccggcccggagggtcccaggggcgggc

SEQ ID NO: 11437 - RNA, 1992 nt, Homo sapiens
  source 1..1992: mol_type = other RNA
ctgaatagctgggactacaggtgcctgccaccacacccgggtgatttttgtatttttagtagagacggggtttcgccatgttgctcaggctggtctcgaactcccgacctcaagtgacttgctcaccttggcctcccaaagtgctgggattacaggtgtgagccactgcacccagcctggcagtcaattttaagcctcctatttcccaggttttagcttaataatcctcattagtttttcagatttttgtcagtcttgttttggggctattttgccttagtgggcctaaacagaatattaaaatacattaataatccatactgagagtagagtataaatgggtttctcactccttagggacacgagtggaaacaatacatcccatgaacacaggtgaatgtccctggttatccctgagctgggcagtttcacacaatcattttttctctgaggccaaagtctgtggtttgatcatcttagcagcttccagaacagaaagtaggtttactttgtctccaaattctttttctcggtgctcaagaagaatgccctgctttcctgatcccaccacgaaaactcccccaaggatgaagccttctccttccaggtttccagagaagcctccgttccaggctcggaagaagttgtaccacactcccagacggataaatcccataaacatcatcttccgcctttgtggaccatagaactttttcttttcatccaggaagatttctcctttgaaataaggctggaaatccttcacttcagtcctgatgtgctcctttaccactgcatagagggggacgcccagctggtccaacatgcttttcagggaggacagatccgcagcttcctctcgacagaggaaacagcctggcctccgcacggccataatcacagctccatttttttcccatagctcctttgctttgaaagtccttggttccttctccagtgttttcaggtctatatcctccaggtactccagggccgctttctggggcttggacagaaacacgtctgtgttggcaagcagcaatgccaaggcagcagcccccagggctcctgcaccaatggaccacatccccatggtgaagaaacttgggtcctggaggaaagacatttctggggctggtccagcagggcggcccccgggcccatgctccagggcagggccctctcctctgttctttgtcccaacaattcgcgaaggttggcgccaccggcgtcactcaaggcttgcgggcgtggacagagggggccctagcccgccgcagcagcgccgggtccccgtctccgttctccgacgtctgggcgcagggtttttccatcggccgccacgcagggtggcggaagggtcgtcgtcctcggagggagcgccagcgctgcggcggctcctaagaaagttggcgcgggcccgaggggcgcgcctcaccagcccagcacccaccctaccggccctgcactgcctcagtttccccacctacgccgcggcaggccccgcctacggacatcacgtgcctcgcggagccccggcgcgcagcacctacctcaagtgcctcccttctgccggccttttaccgccccgacgcccgggcgctaaggggccaaaccgcccggcccggagggtcccaggggcgggccccgcgcttgcgcagcctctagcctgtgctgcatcgcgcgctaccgcgccaccgccatgtgacccgccccgccccccgtgggaggagctccgggcctgcccccgactcgccgacctccgggccgcggtctcctagctccggtggcgctcgggcgtgtgccccagcggtccttttacgcacagcgctcggtcggtccactcctcaagtccgcgaaccgaggccccgacgcgttcttcagggcgctgcctagggcaaaagaaggcgctggacacccctaatggagcctggaagcacctgtcctgcagccgaggctggccaacttccttccaatcttcagcctggtttt

SEQ ID NO: 11438 - RNA, 1256 nt, Homo sapiens
  source 1..1256: mol_type = other RNA
ctgaatagctgggactacaggtgcctgccaccacacccgggtgatttttgtatttttagtagagacggggtttcgccatgttgctcaggctggtctcgaactcccgacctcaagtgacttgctcaccttggcctcccaaagtgctgggattacaggtgtgagccactgcacccagcctggcagtcaattttaagcctcctatttcccaggttttagcttaataatcctcattagtttttcagatttttgtcagtcttgttttggggctattttgccttagtgggcctaaacagaatattaaaatacattaataatccatactgagagtagagtataaatgggtttctcactccttagggacacgagtggaaacaatacatcccatgaacacaggtgaatgtccctggttatccctgagctgggcagtttcacacaatcattttttctctgaggccaaagtctgtggtttgatcatcttagcagcttccagaacagaaagtaggtttactttgtctccaaattctttttctcggtgctcaagaagaatgccctgctttcctgatcccaccacgaaaactcccccaaggatgaagccttctccttccaggtttccagagaagcctccgttccaggctcggaagaagttgtaccacactcccagacggataaatcccataaacatcatcttccgcctttgtggaccatagaactttttcttttcatccaggaagatttctcctttgaaataaggctggaaatccttcacttcagtcctgatgtgctcctttaccactgcatagagggggacgcccagctggtccaacatgcttttcagggaggacagatccgcagcttcctctcgacagaggaaacagcctggcctccgcacggccataatcacagctccatttttttcccatagctcctttgctttgaaagtccttggttccttctccagtgttttcaggtctatatcctccaggtactccagggccgctttctggggcttggacagaaacacgtctgtgttggcaagcagcaatgccaaggcagcagcccccagggctcctgcaccaatggaccacatccccatggtgaagaaacttgggtcctggaggaaagacattttcctcctgttggaagtgcccactctttcatgaaagtaggaggttgtgtccggcgcgctggctcacgcctgtaatctcagggctttgggaggatcgcttgagcccaggagttcaagaccagtctgggca

SEQ ID NO: 11439 - RNA, 1273 nt, Homo sapiens
  source 1..1273: mol_type = other RNA
ctgaatagctgggactacaggtgcctgccaccacacccgggtgatttttgtatttttagtagagacggggtttcgccatgttgctcaggctggtctcgaactcccgacctcaagtgacttgctcaccttggcctcccaaagtgctgggattacaggtgtgagccactgcacccagcctggcagtcaattttaagcctcctatttcccaggttttagcttaataatcctcattagtttttcagatttttgtcagtcttgttttggggctattttgccttagtgggcctaaacagaatattaaaatacattaataatccatactgagagtagagtataaatgggtttctcactccttagggacacgagtggaaacaatacatcccatgaacacaggtgaatgtccctggttatccctgagctgggcagtttcacacaatcattttttctctgaggccaaagtctgtggtttgatcatcttagcagcttccagaacagaaagtaggtttactttgtctccaaattctttttctcggtgctcaagaagaatgccctgctttcctgatcccaccacgaaaactcccccaaggatgaagccttctccttccaggtttccagagaagcctccgttccaggctcggaagaagttgtaccacactcccagacggataaatcccataaacatcatcttccgcctttgtggaccatagaactttttcttttcatccaggaagatttctcctttgaaataaggctggaaatccttcacttcagtcctgatgtgctcctttaccactgcatagagggggacgcccagctggtccaacatgcttttcagggaggacagatccgcagcttcctctcgacagaggaaacagcctggcctccgcacggccataatcacagctccatttttttcccatagctcctttgctttgaaagtccttggttccttctccagtgttttcaggtctatatcctccaggtactccagggccgctttctggggcttggacagaaacacgtctgtgttggcaagcagcaatgccaaggcagcagcccccagggctcctgcaccaatggaccacatccccatggtgaagaaacttgggtcctggggctggtccagcagggcggcccccgggcccatgctccagggcagggccctctcctctgttctttgtcccaacaattcgcgaaggttggcgccaccggcgtcactcaaggcttgcgggcgtggacagagggggccctagcccgccgcagcagcgccggg

SEQ ID NO: 11440 - RNA, 50 nt, Homo sapiens
  source 1..50: mol_type = other RNA
ctgaatagctgggactacaggtgcctgccaccacgccagctagtttttgt

SEQ ID NO: 11441 - RNA, 7704 nt, Homo sapiens
  source 1..7704: mol_type = other RNA
ctgaatagctgggactacaggtgcctgccaccacgcccggcgtgagccacagcgcccggcccccatttgaaattattctttggcaaaatatgtcattaaaacccaaaatgagttaataaaaagcggactcttcccagtttcagtcagctcaaactgcagaacttttgctctcacttgagcttatcatatagctaaagggaaatcagaaaatgctatatacatagcagacatgctatgtatatatacatgcctttgcagtccacaattttggcatgttatggaaacaaagagggtttctcacttctagtggagcccctattaaaaacagactcaagtggatgaacttgctactatcctgttgccatcacaaattggtataagttccaagctatcttgagtaaaggtgaaaaataaataacaaattcttataagattgaagcccatacatggaaagctgaacctgaatatcaagggactgccctggcagattttcatgctaaatcagatagtgctgaaacagttaggatgtgcaaattgaatgaatgccactagattgatgacctttatgatgacccatctaacagtgcaatgcacctgatgtggaaaaccaaaattgttatctgacagacgtaaacataatgttaagcgtgaactcatggagagcctagatggccccctggtccttcctgagcccttgaaacttctattgttaaaagctttgcacttggccaggcacggtggctcttccctataaccccagcactttgggaagctgagctggactgacagcttgagcccaggagttcaagaccagcctgggcaagaggataaaaccctctctataaaaattacaaaaaattagctggggatggtggcgcacactggtagtcccagctactcaggagactgaggtgggaggactgcttgatctctggaggtggaggttgtagtgagccatgattgcaccactgcattccagcctgggtgacagagtgagatcctgtctcaaaacaaaaaaacaaaaaacaacctctgcacctcacaaatgagcaagatgatccagattataaaaaatactgatagtgtgaccactgtaaaatgctgaaatgggttataaccaatatctggtttgtcaaacccataatccagggaagataataaaaactccaagtggtgtatttccaccaacacctgatggaccatttgaacgcttacagatggacttcattcaactgccaccctcaattaagtatcagtatgttcttgtaatagttggcatgttttctggttggatagaagctttcctgtgtaggagagctgatgctatggcagtagctaaggagttataagaacatgtgtttcctttatggggcatctctggaaaaatctccagtgacagaggaactcattttattggacaaactatgaagcagctaaataaagtgttagaaacacagtggtactaccattgtccctttcaccctcagtcttctggaaaggtcaaaaggacaaatattttaaaactaaaattggcaaaattaactgaatcgattggattatcttggccaaagataccaccattggctttgaatttcatttttttctgatctctgaagaagaaagccaaccattgcctttggtcagcagatcagatccattcctacgacagacacagattgacccctatgaaatagttactagaaagcctgtgctcctaacagaacttcacgtagttcctactctcctaaatgctgatgccactaaatactacaaagctgtaatgcattatgtcacactgtattttgacaaaataaaataaactttctgtgacccacagaggaccatcaaagccttcacaatctgtaacctgagactaggtcttctggagatggtatcagagaaaaagtgcccttaaacctcacagaaagagacaataccaagttcttctattacccacactgtggtaaaacttcagggcttcgaaccttgggtccacatctcacaactcaaaaggacctctccagactcctggaactacacacctgttggagactttaaggtaaagctaaccagggaagtttttccccagaagcagatcacgtcctagacatgaacagctttccctagatgtggatgaagacttcactgcaatcgcaaaaatcttatctttctccctctctttcctattttctgtccgcaaatcctttccctttctttatgggaaaatccgtgggaccataatctggggccggctttagcaaaggctaatgctctagcaagaaactggagttcctgttgggtttgtgacttaacgctcaaatcaggaaacgattccattaatgccagtatctctccattttcccaataagtcaccctgaaaccccaaaggaagagtggaatgctaacctttttttttttttttttttgagacggagtctcgctctgtctcccaggctagagtgcagtgacgtgatctcagctcactgcaacctctgcctcccaagtttaagtgattctcatgcctcagcctccctagtaggtgggactacaggcgcatgccgtcacacccagctgattttttgtattttatagtagagacagggtttcactgtgttagccaggattgtctcgatctcctgacctcgtgatccgtccacctcagcctcccagagtgctgggattacaggcgtgagccaccgcatccagcagctaaccttgatattctaaacaccactactgcttgcttccctacactcattggaagtggtaccctgaccttttcaattaataagtgccaatatggaaaaaaacctgtccaggtaatgcctatgcaaggaacactgcctacacctatgctttcaggcaccacatattcaggacctgggaactacctatgtggctccaagcgattgcttatataatgtcactgggttaaatccagtagggttccttctcactggctgtggttatgcacccttacagcatgctataaagggaccacataaaaataagttgcccactggaccttgtttaggagctgtgcagacttatgggggaacataagtgacccctgctcaaatgctaccaggtggcccccactttccagcttcagagggtacatattaggtctgtggataatttgcttactctgtcctgacttcagatcttgctgtttcacctgattcatgctcaccttgcaaacagctttccctgaaagtccccataatcagaggtcaaagactaaaatgaataccaaccttgaaacagatgattagttagtttcccctgagcaaatattccagtggagttcctgcggactcacttttggcggcagtgaggtgccaactgtatggaaattaaagttaatgctaaattgaaaagaattttgtagcacagagattcgcacaggtagaagccacagatggatggatggatggatggatgggtggatgatggatggatggatggatggatggatggatggatggatggatggatgggtggatggatggatgggtggatgggtggatggatggaaggatggatggatggatggatggatgggtggatgggtggatgagtggatggatggatggatgggtggatgggtgggtgggtgggtggatggatgggtgggtgggtggatgggtggacgggtggacgggtggacggatggagggatggatggatggatggatggatggatggatgaggccacctgtgttcaacaaaaacacgtaatggaacttcatgcagctttagatttcctttgcccagctaggagcttgtgtatggtgctgaacaaaactgaacgctgtgcttatctttcctgattctactactatggagagcttcaaaaggcggtggtggctgccgcttctgtagatactgccaccaaacacatcaaggatatttctcagggaaaaggaacacataatgtgtttgcaggagcagctagtggttggtttgcaggcatcctgaatggtagacagcaagcttagctgttcaaggttttctaatcttcatgtttcttttagtgggtatcccaatcaccatgacttgtgttaccaaaagctaactaaaaaatcaaacactttacaattaaggtacttcatagtgaactatgtccttaattgccattataccctgaacaggctatgagcagcagagcttgcacgctgttgaactatttttatcgtctgaacttgagttgtttgattccaatcagtttggtttgtggagactcatattaagggatgcattccagtttcttggtattacactcctgatagccatcctaaggtccccactgatgtgttgtagtcttaagtacaccaatgcagtcatcctttgtacctcaaatggtctcattacggttagagtaacagaaacatgaagacatacagaatccgctaactgatttaacattgtaaactgtgagttccataatgaggtcaaatagtgacagaaggtagtgtcagtgcgtgggattttggtcaatctctcaaaattaaggggctgagcaaaatgagggacactgtgaagctgaattaagtctggcctaaagctgcctctgtacacagtgaattgtaacttaacgtgtaaacaactcgtaacctaacctaaaagtatgttcttctaacaagtagccgaattttagccaatcacagcagccaaaccttcagtcaatcgtcggctgaaggctgctaaaacatgttcaggtaaggcaaatgccagactgcagccaatcaggcaacctaagttattttcgtttctctggctataaatgtagcctacacacattgtggggctgagcattctgaactgcttttggtgctaagtactaaccagttcacgaatcttttttctgctcaaaaacagaacatactttttaaacttcgttaaagttgtctaaggtttttttgccttcaagccctgaagaacaaggagttcatagaacaaaggagaaaagtctcttagccttccaatgacaaaatgaaaagctgccagcaaagtttcaaaggctactctgaaacccaagtcattcttaaaattttacataaaagcccataaatcacttcttactgcagaaagtgaaccagcactttcaagaacagtgattcttcaaatggcgcccaagggcacagcagccactattccaaagatcacactcgcttctggacttcagaatttcccaccctccttgcggcttgttgaactgtttttatcatagttcctcttcttacactggtcacggtgtggaactgaggcatgctgggtaaatgtcaaatgaaatgaaggcacacaatctctattctcaactagacagcaaattgaggtgcacagctcctcttaaaaaaaaaatccatttgtggttgttgatttagtggtccctaacagacaacaggctcctctttgcctgtaccgataataagtgtcagtacagagccagtccttcaattgggctgatcgccaagcactggagaactatggaatgtgcactgatgagaactccagaaattcagtccaacttggctttcactggggaaaaattgggtccagaaaggctgagtgatgtacccaaggccatcccgttggctggtctgctattcctgtccttaggatcacataatacaatttttttccatctttttacctagattcacataagggaaatcctctcccagagtcatttcttatctacccagaaggaatttgcaccctttcaacatcctgggccaagtggtggcgtttcagttcatgtgaatccatgtaaagtactatgatatcgacgacagcctcaaagccaggtgggaggaggaacccacaactttgtctccactgacatctgtatgttatctcattgtcattcatgattccagctattttcctaagttccaaattttctatgactgtcatctggggttttgaaaacagcacctagaaacagagcctagaactctggcctgttctgcttataaattaataaataaaatgcagttctgaggtcaacacctagctccagttgactgtcgtcccagggacacaggctccttccttcccctgacttctgtaaacatgggcactggcacagttagtacgagagcagcagcttgtctccagattagaggggaaaaacccagccttcactttttctgtttggtgggtgaatatcagttattctgtagtcaagagaggctggcaggccaggcctgggctcagggaaaggcagggaggtcttcagaaagctccttgctaggatggccaggttcatcctagcacttcacactcccatggctgggaaaggcatctccgaattaggaaaccacctccctttaaaaataatggccctggggtcagagaggcagagattgcacaaggccacaagtcacttaggtggagctggggctggacaatgcaggacaggaacaaaggcttgctgtgtcaccactcagaagctgcccacatgagaagggcatgacgtcaccagactgtttctggactgggagaccttgaggctctaggagtatttctgacacctacactggttcctcaggtaccgggacctgtagtggaggattgagcccactgagcatctcactgtacaggtaagagaagggaaagctggatccacattccagcctggaatgagccagacactatcctccccaccctctgtctcacccacctccctgcttcggcttcacggccacctcaccaggaaggcttctgcatggttcttggccttgcccaggccctgctcttgaaaggcaaaggaggggaaaagggaaatgctgccatgtggctcttgccccaggcccagtctggcaatgaagcagcagcagtacaactatggtcttgacaggcaggtggcaagcaggagagctccagcctaggagaggagctccaagagcagtttccagatgtgcacggtgccaggctcttcaaaggtgggtcctgcaggggcaatgctggctgccaagaggaaaacctcccgctggttatcgatagcctgtagacccagctcccgctgcagctcccccatactcatggcctcgctcaggtcctgcttgttggccaccacgacgacaggcaggtcagggtccttgtccagcagcttgtgcagctcctgtcgggcccagggcagccgcagtcggtcagccgagtccaccacaaacaccagcacatccacctcgctcacaaactccttccagtagaagcgcaggttctggctgcccccaatttctagcaggtccacctcaaagtccttggtgggcagacgcacggagttgaagccccaggtggggatgtggccttccagcggtggcttccccgacaacacgcgcaggaacgtgctcttgcctgcgccatccagccccagcaccagcacctcgcgctgttccagctcctccagcgccggctcctcgtcctcctcgtcctcggggtcccactcgtcccactcggggaggcgggcagcctccgcgccccaccaggcctctccccggtcccagcgccgctctcggccgcggccgaagtaggtcttccagaggatgaagagcaccgagcccagcaccgccgcggcgccgcccagcgccagcaccaaggggcccagcggccgcggcgccatcgggccgggcgagggacgcaggtgcgggttgcacaggccgagcccactcgcccgccgaagatggccccgctgcgact

SEQ ID NO: 11442 - RNA, 1222 nt, Homo sapiens
  source 1..1222: mol_type = other RNA
ctgaatagctgggactacaggtgcctgccaccacgcccggctaatttttgtatttttagtagagacagggtttcaccatattggccaggatggtctcgatctcctgaccttgtgatccgcccgcctcatcctcccacagtgctgggattacaggcgtgagccaccgtgcccggccctggatagcttttcaatatggttagaagacattttcattttacttttctgttctcttctccatccttccttcttccctcccttcctctatctttcctttttaacacaaaaggagaaagcactaacagtgttggcaatctatatgggacctagatagaagagcataacacatctaattaaattgctccctctcttggctcagactgccatgacaaaataccataggctgtatagcttaaacgacagacatgtgtttctcatggttcttttccagccttcttttcttccagcctcctcagatgggaaccctctcctctgcattcccactgttcgtccccatatttgtttcttttttctttttgagacggagtcttgctgtcacccaggctggagtgcagtggcaggatctcagctcactgcagccccacctcctggattgatgcagttctccagcttcagcctcccaagtagctgagattacaggcacacgccaccacatccaactaatttttgtatttttagtagagacggggtttcaccatgttggccaggctggtcttgaacttctagcctcaggtgatccggccatctcggcctcccaaagtgctgggattacaggcgggagccaccgcgaccggccccctatacttctttcaaagcacccgagttcaggaggggaaatggcatggtctgcccaggtgctgttgccgccaagcaggagccttgcgctccaactgcgtccctcgaagtcttcaggcaaaagcgggactggggagtccagtcctgtggcccagccacatttcctcgcgtagaacgttggacaatgttttctacctcacaggaccatccaaatgactgcgttaggtattcccatgaaatgtacgatgagtacaccctattctacagaagcaaaagctgaggctcagagacgccaagaggtttgctggggtctcgcgactaagcggtcccaacacccagacaccctggctacccggggactgccggtcactaccgggcgccgaaaagccgccggctccttccgccagct

SEQ ID NO: 11443 - RNA, 1361 nt, Homo sapiens
  source 1..1361: mol_type = other RNA
ctgaatagctgggactacaggtgcctgccaccacgcccggctaattttttgtatttttagtagagacgggatttcaccatgttagccaggatcgtctcgatctcctgacctcgtgatccactcacctcggcctcccaaagtgctgggattacaggtgtgagcgaccgcgcctggcctgcatcatttctgttttgaaatatagtcatggcttcaagatttaatgcacatacacccctcatgaaagcttttttcatggaatcttcaaagtgctctttttcatgttgcattctttgaatctcagcttttgcattttccaaagctccagataacatagcaactttggcttcataatcattggaaatctggatacaaacttcttcagctcttgcttgacaagctctttctaccacatctttccactgcttttgcactacggaacgccagactttccagactttcttcagtaaagttctctggtagtactggtcagctagtttaccttcataaacatcctgtctggctctgacatggccgattcgccagtggaagaatgttctcatcaactctatcttttccttttgcttgcctatggcatgagacaagctagaaatcacctcatcttttctcccaatggagatttcaaaggttttttgcagctccttcaattcattgatctgattacacagttgttttaaatgtgctgcatgtttttctttctcttttctcatttccattcggtgccagtcaataaaattaagtctccatttacttagttcagatatgatgtttgtcttaagacctgaactccaaagatcaagcacattttccatcttctgaaggttttcatcagaaacaagaaaatcgctcacaagtatttcatgggcatctgtatgactagaatttgttgctggtgaggaagagtcagctaaaagatgtgaactgaaaaaatccatgactgggtgagaaggcttccttggcgataacactggtgatgactcatctgtctttgaatgacttgaaatatggaaatcacatccttttccaacttctattgcagtttctcttacttcagagttatttccttgactatgaagaatatcatgaattgtagaaattctgacatctggcaccaattctcccttaggatgagatgactgtgaagcacagggttcaatatttggagtcactatagcataatgaagcagttcttcatattcttccgtcgccgctcgcgaccaaatcccgactcctcgctctgcgcctcttagccgcgtcgcagctgcagtgtcagcaagtgcagcctcagcaagcacaaccgctacctagacggcaacctgacagtttcaaactgcagggaggaa

SEQ ID NO: 11444 - RNA, 1501 nt, Homo sapiens
  source 1..1501: mol_type = other RNA
ctgaatagctgggactacaggtgcctgccaccacgcccggctaattttttgtatttttagtagagacgggatttcaccatgttagccaggatcgtctcgatctcctgacctcgtgatccactcacctcggcctcccaaagtgctgggattacaggtgtgagcgaccgcgcctggcctgcatcatttctgttttgaaatatagtcatggcttcaagatttaatgcacatacacccctcatgaaagcttttttcatggaatcttcaaagtgctctttttcatgttgcattctttgaatctcagcttttgcattttccaaagctccagataacatagcaactttggcttcataatcattggaaatctggatacaaacttcttcagctcttgcttgacaagctctttctaccacatctttccactgcttttgcactacggaacgccagactttccagactttcttcagtaaagttctctggtagtactggtcagctagtttaccttcataaacatcctgtctggctctgacatggccgattcgccagtggaagaatgttctcatcaactctatcttttccttttgcttgcctatggcatgagacaagctagaaatcacctcatcttttctcccaatggagatttcaaaggttttttgcagctccttcaattcattgatctgattacacagttgttttaaatgtgctgcatgtttttctttctcttttctcatttccattcggtgccagtcaataaaattaagtctccatttacttagttcagatatgatgtttgtcttaagacctgaactccaaagatcaagcacattttccatcttctgaaggttttcatcagaaacaagaaaatcgctcacaagtatttcatgggcatctgtatgactagaatttgttgctggtgaggaagagtcagctaaaagatgtgaactgaaaaaatccatgactgggtgagaaggcttccttggcgataacactggtgatgactcatctgtctttgaatgacttgaaatatggaaatcacatccttttccaacttctattgcagtttctcttacttcagagttatttccttgactatgaagaatatcatgaattgtagaaattctgacatctggcaccaattctcccttaggatgagatgactgtgaagcacagggttcaatatttggagtcactatagcataatgaagcagttcttcatattcttcctgaagattcgaagagacagaactgcctcgactggagtcattttgcacaactggaagtgagtatttctcctcatctgatgacattctgcacaaatgctcgtcgccgctcgcgaccaaatcccgactcctcgctctgcgcctcttagccgcgtcgcagctgcagtgtcagcaagtgcagcctcagcaagcacaaccgctacctagacggcaacctgacagtttcaaactgcagggaggaattaaggaccgccctgggcattggtcctttgtttcagcaatct

SEQ ID NO: 11445 - RNA, 7485 nt, Homo sapiens
  source 1..7485: mol_type = other RNA
ctgaatagctgggactacaggtgcctgccaccacgcccggctaattttttgtatttttagtagagacggggtttcaacatgttaaccaggacggtctcgatctcctgacctcatgatccgcctgcctcagcctcccaaagtgctgggattacaggcgtgagccaccacgcccggctccggttaccttttaagcattttgtggggcagggggagatctgtgcagggggaagcatattacagaagcaagaaacaaagacagttattcagttgagacatgcattacatcattttttacttttcaaggaaaaacatgttttatgacttgagtttatctgcctagtgaccttgcagctgcacagctagagaaacagggtcttcacaatgcctgggaaagggagagagataaggctcactatccacagaaaaacaggcagttaatttttaaaggactttagctctttctcttcctcagggtgaatggggttttcttacatacaactgagtttttgcttacacattctttaatttcttttaattcctgttttaactctctcacccagactggaatgcagtggcccgatctcagctcatcggaacctctgcctcccaggttcaagtgattctcctgcctcagcctcctgagtagctgggattgcaggcatgcaccaccatgcctggctaatttttgtatttttagtaaagatggggtttcaccatgttgaccagactggtctcgaactcctgacctcaggtgattcacccgcctcaacctccaaaagtgctgggattacaggcgtgagccactgcacctggccacgataaatgttcttgcttgcagttttatcatggccttggcaggttcaagtttgctattatgctacctaaagatgtcaggaaacacaggaaatgtcttggcagccagtttctgggggtttccagcgttcccgtggagaggagggactcacggaggggacgctggtgctttagaacacatgtgctggaggaactcctttctctgttcacatttcaccttcctacatccccagggagaccctgcctgggtcaggcagccccacccgacaaggaccacctggattacgcagcttttcccacaaagcccacctcactcagtcagccatgggccatttccttcaatgcatgcagctcaagctggggcaactatacgcagaaagaacctgtggcagcttcgaaagaaagtttcctgatataattccaacaaaaggcagcatacattactcagctctgcagggagactaaagccagcccgggtcccggaaggcacaggagtgtttggacggtggctctggctgccggagacgccacaagagccttccctccctccctcccacacgaacagcagacttgcgacacggtctgatggccctccccatcttccctcacatgggcatcttccctcctaaaatctctgcccatttaatcctatcttggcatctgcttctcagagtacccatttcctcagaaggaggctttgggtctcagataccaccatccctccagacaccatggcctgtgtgtagacaattcaatgccgtgggctacacatggtggaggagctgctgggcgatccagagaggagagtaactgattcttcctggaggcctagaaggtcaagagaggacaggaaatggtggtgttttgggagagccatgaaggataagtgggagggaactgacattcctaaaaaagaagtgcaggggccaggcccgacagctcatgcctgtaatcccagcactttgggaggctgaggcgggcagatcatttgaggtcaggagttcgagatcagcctggccaacatggcaaaaccccgcctctactaaaaatacaaataaaaatgaaaaaactaacctggcgtggtggtgggtgcctgtaatcctagctactgcggaggctgaggcaggagaatcacttgaacctgggaggcagaggttgcagtgagctgagatagcaccattgcactccagcctgggcgacagagcaagactgcatctcaaaaaaaaaaaaaaaaaaaaggaggtgcagagaccccagcagttcagttcagcatagccagagtgtagacatgcacagggcggtgatccaaggtgaggctggacacagcccacagcccacagtctacagggtgaggagcaacacaggagaccacaggtccctccctcactgtggccagtccttagcctgagcaatgacagagagttcagtgacagtcaatggacagcagcctttccccaacactaggatcccaaagagcttttgttatgtggttttatctttcaatatttgccctgttagatattaaaacagagaacttttctttttaagatgaagctggggctgggcgcggcggttcaagcctgtaatcctagtactttgggaggccgagttgggggatcccctgaggtcaggagttcgagaccaggctggccaacatagtgaagcccctgtccccactagaaatacaaaaatcagctaggcgtagtgtcacctgcctatagtcccagctactcgggaggctgaggcaggaggatcacttgaacctgggaggcagaggttgcagtgagccaagatcacaccactgcactctaacctgggtgacacggtgagactccatctcaaaaaataataataaaataaaagatgaagctgggctgggctcagtggctcacacctgtaatcccaacactttgggaagccaagatgggaggatcgcttgaggccaggagctcgagaccagcatgagcaacatagtgagacctcatctctaccaaaatacaaaaaataaaaaatagtcaggcatggtgatgggtgcctgccatcctatctactcaggaggctggagtgggaggatcatgtgagcccaggaggtcaaggctgcagtgagccacaatcacaccattgcactccagcctgtgcgacagagcaagaccttgtctcaaaaaaaaaaattgttttttaactaaaaacagatgaagctggaaggccagcctgtaatcccagcactttgggaggccaaaatgggtggatcacctgaggtcaggagttcgagaccagcctggcgggcacctgtaatcccagctactcgggaggctgaggcaggagaatcccttgaacctaggaggcggaggttacggtgatcacaccactgcactccagcctgggcgacagagcgagactctgtctcaaacaaaacaaacaaaccaaccaacaaaaaaaatggcagaacagctcaaatgctaagccaaagactgggggctttatcctgtaggcaagagggagttgttgaaagttttgagcaactgagtcccgtgaccacatttgcatttttggaaacattaccaagtcaggattaaaggctggagggcaattaggaggccttgcagtaggtcacatgtcttttcatgtggatttaatgaggaaggagtcagaatataacagttttattaatggtgttggattttacaaccaaataatcccttagctatattgttttattttctaacatgaaagagcttctaccgttaatcctctcttctgtctcctgaagccagggctccacaggccttcctctgggagacacacccaggtgtgccgccttcccctgccagatcctcaggcctttcttacccaactcacaacttccctttcacccttagtcccatacccaccatctcccgagaaaacctccgcaatgggctgccggggccccaggcccttccacccatcccgccagcacaccctccccgtgaaaatgagtgaccccaggccagcgtcttccctcaggagagaagcctgtctggatccccaaaggcctctccctccagggaagagggactctcactctggcctcagtggttactccagagcccaagaaatgccctgtgcgctaaaaccaaagaaggtgtgaaccagcaagtaagtggggagcggccagttctgggacatctagttgggggccttctcttccccatgagcagcagggaccagtgtgaccttggcatcaggctctttctcttggctggcttcctcaacgttcaagacgctcgataaacatatcccagaggcaaagcaagttaagtcgagggttgtttattcacctagaatcagctccagccattttccaatgtcttctttttgttgtttttctggtttttgttgcaacagggtctcactatgttccccaggctggtctcaaactcctggcctcaaatgagcctcctgcctcaaactcccaaagtgttgggtttacaggcatgagtacccagcccttaagtgtctttgctttggtttatgtttgtttgtttccttccactcctggtgcaaaccttacatgtttttgactggggaaacatattttggacctatgcctctacactgacagtgaagagcccaatgggttgtgcactaggtcagggcttcccgcagcgtcagcccctgtggccagcagcgtcacctgggaacctgctagaaatgcacatttttggcagggcgtggtggctcacacctgtaatcccagcacttggaaggccaaggcaggaggatcacctgaggccaagagttcaagatcagcctgggcaatgtaacgagacaccatttctacaaaaactaaattaaaaaaaaaaaaatgagcattttcagccaggtgcagtggctcatgtctgtaatcccagcactatgggaggccaaggcgggtgaatcacttgaggtcaggagttcgagaccagcttggccaacatagtgaaacccctactaaaaataaaaataaatagccaggtgtggtggcgggcgtctgtagtcccagctacttgggaggctgaggcatgagaattgcttgaaccctggaggcagaggttgcagtgagccgagatggcaccactgcactctagccttgagtgacagagcaagactctgtctcaaaaaaaaaaaaaaaaaaaaaaaaaagaaataaaaaaaagaaatgagcatttttgacctgtccaacctactaaatcagaaacttagcaccctatgctttaacaagtcatggctaagggctttaaaaaggtgattttaatgcatgcctaaggtggagaactaaggagaaggcttttgggtaaggtgaatctggagcgggggacccaaggcctaaggaggaggggagtgtgaggcaaaaggagccccttatctacaggttctcaagctcctcccatcaatcccccaacctggccctgtccctccctcgctcaaccttagtttcttcctggaattctcaggcctcctggttcccaaattctgatttccccactgacctgactccagatctccctaccccactgggtcttgtccccagcgtcactccaacccctcaccagcagtccccaggccatgccaacccccacacttttttttttttttgagacagagtctcactcttgtcacccaggctagagtgcagtgccgcaatgtctgctcactgcaacctccacctcctgggttcaagcaattatcctgcctcagcctcccaactagctgggattacaggcgtatgccaccgcgcccagctcatttttgtattttcagtagagaggagtttcaccatgttggccaggctggtcttgaactcctgacctcaggtgatccacccgcctccgtctcccaaagtgctgggattacaggcatgagccaccaagccagtcctaccccacgcttgtcagtattctgggagatcccccagttcccagccccctgggccctggcaacccgctccccacccttctcccgtcagacccgaccaaggagacctaagcttcaacccaggcccccgcgcccctccactacccgtccggcggctcaggcctcggcgccttcgggacccacgagcagcagcggctgggcattcttgcccttgtcgtgccagcacacgtcgaagaaggggtacacgggcctgggcaggcgctcgtggaaggcaaaaagcggcacgagcgcgtcggcgtcgctggcatcgtagaaggagaggacgccgtcgccgaagctcaggtaaaggccaatgcgcgtgggccgcctctcggggctgcgcagagcgcgcggctccttggcctccacgtgtgcctccaggatcttgccctcgcgcagccccagcagccacaggccctgcgagggcaccgcgtgcaggcgcccgcggcggggggcctcggccgcgatcacgcccagcgcccagcgcggcttgtcgccaacatccacctcccagtagtgctcgccctcggagagctgctggtgcgccaccaccgccaccgccttgtcgaactggcgcgggtcctccccggccggcggcgccttctgctccgagcactccacgcggcggccagaggaagacaccaccaggctcgggtgcgcagagctcgggtcaaaggtcagctcctccagcgctggcatcagagcccggaacatcttcctccacacctggaatttgaagtcatctgagataattggcagctggatgtccagacgggcgggtgggggagactctgccaggatcttctgcagcctgctggtcaccaggcagtatttcatgaggaactcagtctgcggcttgtccgccacctcctccaggaccttctccatctgccgcagctgctccaggtaagagttcaggctccccagctcccggcgcaaggcgacccctgcctcaccccgtacacgctctgcctcgcggtccaaggagccctccagtgcagccaggaacacccgcatcttgcccagctgctcccccacggccccccggaactgacgcactgtctcctccacctccaccagctgatgctccagcacagccacactcttctccttgcgcatgcatgcctcctgcagctgcagtttctgctgtggcagctgtgtcttgaggcgtgcgtgggcctcggcggcaggcaggaggcgatgaccgcggtgcgagccgagtgaggcgcacactccgcacaccagcgcgcggtcctgctcgcagtagatgctcagcgggtccaggtgctcctcgcagtggccctgcggcacctgggccagcccctccaccaggcgcgccagctgcaggttggtgctgagtgcctgcggccgcgtgggggcctggcagcaggggcagagaacggtgccatccgccgccggctccccggccacgcggcctaggcaggcgcggcagaaactgtggccgcactcggctgtcacgggcgcgtcgaacagctgcaggcacagcgggcaggacagctcctggtgcaggaggccgggcgcagccgacatggcgggcaggtctggttggagatcttaggctgaaagagtctcgaaggaggaccggtcagggttgagcttagctggactggggtcagggctgggtccaaggatctgagacaagcagcaggctccaagcaaggacagggactcacaggggcagctggcagtggacaccacgcgtgatgggcacacagt

SEQ ID NO: 11446 - RNA, 4229 nt, Homo sapiens
  source 1..4229: mol_type = other RNA
ctgaatagctgggactacaggtgcctgccaccacgcccggctaattttttgtatttttagtagagacggggtttcactgtgttagccaggatggtctcgaactcctgaccttgtgatccacccacctcggcctcccaaagtgctgggattacaggcgtgagccaccgcgcccggctatgaagactatttttataagtaaataattatgaaacctctgcaagtacatttccctcctcacatttacgttcttagctaggaaacactgggaggtagagacttctctgcctgcaaaggaattctagattctaaagcaaagttgcttgtgggacaaaggaaaaagatatatacatatcttctgtagaaattatcccaaaaactcaggaccactcagggaagacatggaatttaggataaaggcagaccctgggaagcacacagttcagatcactagagagctttggctgctacagaacaggagataggagggaagaatgcaggagggtacatgggaaagcagctgtgaagtgcacactactcccagacatcctcctgaaagagaagttagcactaagataagggtaggtaacaaagtaaggaagaaagggaattaaggtgagagaaaggcaaaagcagaggggaaaccttctcaagaaagggagtaatgctgaagaatttagagagttgagtaaaaggtttattattagtgcagtcaacaccatggaacagcacatacaacacaaccagcaacctgcagagacactagtgcaaagggtagggaagcctttcactgagcttcctggctccatctgagggtaaggacaggacagtatgagccttggttaaggcaggtaggggaaaggggagtggaagaaatgtagtaaccagagtaagtatagcagcgttttcaaattcctgagcacaatgtcccagagctggaaccctactcccctcaagctttccaccccaatcccagtggagccatgatccaactacccagacctgcagcaagctagcctggaataaaattctgagaggaagccattacatggtggggaggagcctttctatctccaaccacactcccacctccatattaaaataatcacacctattatctctccccttctcttactctgccagtcactctagggatcaaggtataccccaggtaacctgaaatggaactgaagtccccaggggggtgtgggtgagacacggcacagcctgtacttagagataaaatttctgatttgcatggtgaagcttagaacccagctatacagctccaaggaaacttggggaagggggagttgccttcaaaatgaatactctaaatccagagttttatgataaggccctggaagggctaggaggaaatttttccagagggcacaggcatcgatgctggactgtcatatccttcacaggaagagaggaagctcctcatttcagttggggttacagaggtttggggcagatatcgtaagttcagccgaggactcccttggctcttcctatattaaagccaaaggttgtgctgaaaaggaaaaaatataaaacacacccccatccctgtcccaccctatccagaacccccacaataggaacatcaaaagaaaagtttcaagtttgatttttttttcttttttcctttcttaaaaaaaaaaaaaggaagtaaataaattaaattgccaacaatgtggctgagatagccatgatcaggccattcttaaaaaaaagaggggggggggcagtaggtggagtttgtgaaatataaacaaacaatggccaaagaaaattatcaaagtaactaactacagtcacagggctagagaggggtctatggaacaattatggcctgtgccacaagaggcagtgccaaccatattttagcaaaagctaggagtagcttcttgctaaacacatcaacccccaacagattaacccctaccctaaaccctggcattccctaattatgaaaacttgtaggaaagaagagctcatctggaaattttcagtatcccaacctgcatactggtagacccagtgggtgcctacacctttaaggtgggctgaacagggatactgcttggcacagaggtccagtctttccctaagggccatcagtgatggccaattaacggcctcactacttatttctagagatttggctccacccttaccatttcttcaggatgtctgctgcttagagtcaacaggcctgactgctctgattccctggttttggaggagagggacgattagagattccttcctctgtcctgatcctccagggaaattgaatctctttgtgctttctgaaaataactggaaccagggaccctaagcaggaaaatggatggaggtgggggctttcccacccagactgataatttatagacattttaggggaatatggcaaagggaggaaatctgggtttcccacctgaaaggctgagcaaactaccccaaggcccttcagtgccagaagggcagggagatgtgtggctcaggtataagccacagtattaagaatggtgggtaggactcaggtcccagctgctggagtgatgggattttctgatttccatctcttcctgatagccagtcgagttctcttatatctcttccacgccatgcgcaaatatcatgacaaggcctggctcttgcaccatgtcatcccccatgtgctggttctcacaggccatcacgacaacagcctgcttgccagggatgcgcttggccacgtagttctcatagtagcgtcggttcatctgtctagtctctagtgtggccagaccctggggccagctacgctcgtgggcattttcaatcagctcgttgacaatagaagcaggacagccactctccaccagggagcgcttgattacagcctggagcacagcatcaggagtcgagatcatccctccccagcgggtcactcttgctggctgaagggagttcacccacagtttactctatgaactgtataggactccagaactgaaagagatcttagacttcacttgtatacttcgcttgtttttgctgcattttagagatcactttcctggacttgcactctgcctcctcttctctgggttgtaagctactctaggatctcgttgtattcaattgtctcctccaggttctgaaggttggggttgacactgcggattgcacgcatgtatgcctttagcagctggatgtctcgcttctgctccgccagctggtgtttgtgttcagctgacgtcttctccagctctgcgatgcgtgtctgctgctgctgtaccactgagcgcaggtgcttaatgcagttatggttgggcagctcatctttgggcatctccaggccacagccctgttcacaggtcacaggccgcttcgggttgtgctcacagtcgctgaggtgagacatgaggttgtcaagccggacaacggcactacagccgaacacagcgttgtcacaggcaatctgcagctttgacaacatgttccgcatgatccgaggtactgggcgcagatgggcgaccgtcacaacactacggtccactggacatgtctgttgctgagagaaccactgggtgatgcaggcgttgcagaaagcatgttcacaatgaggtgcctggtaatcgtgagcttctcctcatacttgccccaggatgatacaactgactctggtctggcaaggctggcagagaaatgacctattgaaggtggcagctttcacatcaaaatgcagagtgcatggctgtatcaaaagctggtctgtactggctcctccaagactccactgcaaatagggcagataagatcttcgtcaacatccccctggaaacgggttacatcataccccatgtctcatcactgaaacccaggtccttccaagtgttggggggcaggttccctgttcacaaggctccaaccccctgatgcctccactcagtgccactgaagagattctcccagtaacccatcttgttggctattctccgactgagtattccttcccagtgacaagctccatcgcccaggggatgaatgtgatgtcacaatcaggagtactcgccctggaagcggcctggagtctccgcaacctgacccagtcggagctgaggccgcagcggccacagtactgccctggtgccgggtcccagcctctcccgggaagggaagggaaaggggaaggaggggaaagaagactcctaccactcgtcgccgcctcagac

SEQ ID NO: 11447 - RNA, 4086 nt, Homo sapiens
  source 1..4086: mol_type = other RNA
ctgaatagctgggactacaggtgcctgccaccacgcccggctaattttttgtatttttagtagagacggggtttcactgtgttagccaggatggtctcgaactcctgaccttgtgatccacccacctcggcctcccaaagtgctgggattacaggcgtgagccaccgcgcccggctatgaagactatttttataagtaaataattatgaaacctctgcaagtacatttccctcctcacatttacgttcttagctaggaaacactgggaggtagagacttctctgcctgcaaaggaattctagattctaaagcaaagttgcttgtgggacaaaggaaaaagatatatacatatcttctgtagaaattatcccaaaaactcaggaccactcagggaagacatggaatttaggataaaggcagaccctgggaagcacacagttcagatcactagagagctttggctgctacagaacaggagataggagggaagaatgcaggagggtacatgggaaagcagctgtgaagtgcacactactcccagacatcctcctgaaagagaagttagcactaagataagggtaggtaacaaagtaaggaagaaagggaattaaggtgagagaaaggcaaaagcagaggggaaaccttctcaagaaagggagtaatgctgaagaatttagagagttgagtaaaaggtttattattagtgcagtcaacaccatggaacagcacatacaacacaaccagcaacctgcagagacactagtgcaaagggtagggaagcctttcactgagcttcctggctccatctgagggtaaggacaggacagtatgagccttggttaaggcaggtaggggaaaggggagtggaagaaatgtagtaaccagagtaagtatagcagcgttttcaaattcctgagcacaatgtcccagagctggaaccctactcccctcaagctttccaccccaatcccagtggagccatgatccaactacccagacctgcagcaagctagcctggaataaaattctgagaggaagccattacatggtggggaggagcctttctatctccaaccacactcccacctccatattaaaataatcacacctattatctctccccttctcttactctgccagtcactctagggatcaaggtataccccaggtaacctgaaatggaactgaagtccccaggggggtgtgggtgagacacggcacagcctgtacttagagataaaatttctgatttgcatggtgaagcttagaacccagctatacagctccaaggaaacttggggaagggggagttgccttcaaaatgaatactctaaatccagagttttatgataaggccctggaagggctaggaggaaatttttccagagggcacaggcatcgatgctggactgtcatatccttcacaggaagagaggaagctcctcatttcagttggggttacagaggtttggggcagatatcgtaagttcagccgaggactcccttggctcttcctatattaaagccaaaggttgtgctgaaaaggaaaaaatataaaacacacccccatccctgtcccaccctatccagaacccccacaataggaacatcaaaagaaaagtttcaagtttgatttttttttcttttttcctttcttaaaaaaaaaaaaaggaagtaaataaattaaattgccaacaatgtggctgagatagccatgatcaggccattcttaaaaaaaagaggggggggggcagtaggtggagtttgtgaaatataaacaaacaatggccaaagaaaattatcaaagtaactaactacagtcacagggctagagaggggtctatggaacaattatggcctgtgccacaagaggcagtgccaaccatattttagcaaaagctaggagtagcttcttgctaaacacatcaacccccaacagattaacccctaccctaaaccctggcattccctaattatgaaaacttgtaggaaagaagagctcatctggaaattttcagtatcccaacctgcatactggtagacccagtgggtgcctacacctttaaggtgggctgaacagggatactgcttggcacagaggtccagtctttccctaagggccatcagtgatggccaattaacggcctcactacttatttctagagatttggctccacccttaccatttcttcaggatgtctgctgcttagagtcaacaggcctgactgctctgattccctggttttggaggagagggacgattagagattccttcctctgtcctgatcctccagggaaattgaatctctttgtgctttctgaaaataactggaaccagggaccctaagcaggaaaatggatggaggtgggggctttcccacccagactgataatttatagacattttaggggaatatggcaaagggaggaaatctgggtttcccacctgaaaggctgagcaaactaccccaaggcccttcagtgccagaagggcagggagatgtgtggctcaggtataagccacagtattaagaatggtgggtaggactcaggtcccagctgctggagtgatgggattttctgatttccatctcttcctgatagccagtcgagttctcttatatctcttccacgccatgcgcaaatatcatgacaaggcctggctcttgcaccatgtcatcccccatgtgctggttctcacaggccatcacgacaacagcctgcttgccagggatgcgcttggccacgtagttctcatagtagcgtcggttcatctgtctagtctctagtgtggccagaccctggggccagctacgctcgtgggcattttcaatcagctcgttgacaatagaagcaggacagccactctccaccagggagcgcttgattacagcctggagcacagcatcaggagtcgagatcatccctccccagcgggtcactcttgctggctgaagggagttcacccactctaggatctcgttgtattcaattgtctcctccaggttctgaaggttggggttgacactgcggattgcacgcatgtatgcctttagcagctggatgtctcgcttctgctccgccagctggtgtttgtgttcagctgacgtcttctccagctctgcgatgcgtgtctgctgctgctgtaccactgagcgcaggtgcttaatgcagttatggttgggcagctcatctttgggcatctccaggccacagccctgttcacaggtcacaggccgcttcgggttgtgctcacagtcgctgaggtgagacatgaggttgtcaagccggacaacggcactacagccgaacacagcgttgtcacaggcaatctgcagctttgacaacatgttccgcatgatccgaggtactgggcgcagatgggcgaccgtcacaacactacggtccactggacatgtctgttgctgagagaaccactgggtgatgcaggcgttgcagaaagcatgttcacaatgaggtgcctggtaatcgtgagcttctcctcatacttgccccaggatgatacaactgactctggtctggcaaggctggcagagaaatgacctattgaaggtggcagctttcacatcaaaatgcagagtgcatggctgtatcaaaagctggtctgtactggctcctccaagactccactgcaaatagggcagataagatcttcgtcaacatccccctggaaacgggttacatcataccccatgtctcatcactgaaacccaggtccttccaagtgttggggggcaggttccctgttcacaaggctccaaccccctgatgcctccactcagtgccactgaagagattctcccagtaacccatcttgttggctattctccgactgagtattccttcccagtgacaagctccatcgcccaggggatgaatgtgatgtcacaatcaggagtactcgccctggaagcggcctggagtctccgcaacctgacccagtcggagctgaggccgcagcggccacagtactgccctggtgccgggtcccagcctctcccgggaagggaagggaaaggggaaggaggggaaagaagactcctaccactcgtcgccgcctcagac

SEQ ID NO: 11448 - RNA, 3847 nt, Homo sapiens
  source 1..3847: mol_type = other RNA
ctgaatagctgggactacaggtgcctgccaccacgcccggctaattttttgtatttttagtagagacggggtttcactgtgttagccaggatggtctcgaactcctgaccttgtgatccacccacctcggcctcccaaagtgctgggattacaggcgtgagccaccgcgcccggctatgaagactatttttataagtaaataattatgaaacctctgcaagtacatttccctcctcacatttacgttcttagctaggaaacactgggaggtagagacttctctgcctgcaaaggaattctagattctaaagcaaagttgcttgtgggacaaaggaaaaagatatatacatatcttctgtagaaattatcccaaaaactcaggaccactcagggaagacatggaatttaggataaaggcagaccctgggaagcacacagttcagatcactagagagctttggctgctacagaacaggagataggagggaagaatgcaggagggtacatgggaaagcagctgtgaagtgcacactactcccagacatcctcctgaaagagaagttagcactaagataagggtaggtaacaaagtaaggaagaaagggaattaaggtgagagaaaggcaaaagcagaggggaaaccttctcaagaaagggagtaatgctgaagaatttagagagttgagtaaaaggtttattattagtgcagtcaacaccatggaacagcacatacaacacaaccagcaacctgcagagacactagtgcaaagggtagggaagcctttcactgagcttcctggctccatctgagggtaaggacaggacagtatgagccttggttaaggcaggtaggggaaaggggagtggaagaaatgtagtaaccagagtaagtatagcagcgttttcaaattcctgagcacaatgtcccagagctggaaccctactcccctcaagctttccaccccaatcccagtggagccatgatccaactacccagacctgcagcaagctagcctggaataaaattctgagaggaagccattacatggtggggaggagcctttctatctccaaccacactcccacctccatattaaaataatcacacctattatctctccccttctcttactctgccagtcactctagggatcaaggtataccccaggtaacctgaaatggaactgaagtccccaggggggtgtgggtgagacacggcacagcctgtacttagagataaaatttctgatttgcatggtgaagcttagaacccagctatacagctccaaggaaacttggggaagggggagttgccttcaaaatgaatactctaaatccagagttttatgataaggccctggaagggctaggaggaaatttttccagagggcacaggcatcgatgctggactgtcatatccttcacaggaagagaggaagctcctcatttcagttggggttacagaggtttggggcagatatcgtaagttcagccgaggactcccttggctcttcctatattaaagccaaaggttgtgctgaaaaggaaaaaatataaaacacacccccatccctgtcccaccctatccagaacccccacaataggaacatcaaaagaaaagtttcaagtttgatttttttttcttttttcctttcttaaaaaaaaaaaaaggaagtaaataaattaaattgccaacaatgtggctgagatagccatgatcaggccattcttaaaaaaaagaggggggggggcagtaggtggagtttgtgaaatataaacaaacaatggccaaagaaaattatcaaagtaactaactacagtcacagggctagagaggggtctatggaacaattatggcctgtgccacaagaggcagtgccaaccatattttagcaaaagctaggagtagcttcttgctaaacacatcaacccccaacagattaacccctaccctaaaccctggcattccctaattatgaaaacttgtaggaaagaagagctcatctggaaattttcagtatcccaacctgcatactggtagacccagtgggtgcctacacctttaaggtgggctgaacagggatactgcttggcacagaggtccagtctttccctaagggccatcagtgatggccaattaacggcctcactacttatttctagagatttggctccacccttaccatttcttcaggatgtctgctgcttagagtcaacaggcctgactgctctgattccctggttttggaggagagggacgattagagattccttcctctgtcctgatcctccagggaaattgaatctctttgtgctttctgaaaataactggaaccagggaccctaagcaggaaaatggatggaggtgggggctttcccacccagactgataatttatagacattttaggggaatatggcaaagggaggaaatctgggtttcccacctgaaaggctgagcaaactaccccaaggcccttcagtgccagaagggcagggagatgtgtggctcaggtataagccacagtattaagaatggtgggtaggactcaggtcccagctgctggagtgatgggattttctgatttccatctcttcctgatagccagtcgagttctcttatatctcttccacgccatgcgcaaatatcatgacaaggcctggctcttgcaccatgtcatcccccatgtgctggttctcacaggccatcacgacaacagcctgcttgccagggatgcgcttggccacgtagttctcatagtagcgtcggttcatctgtctagtctctagtgtggccagaccctggggccagctacgctcgtgggcattttcaatcagctcgttgacaatagaagcaggacagccactctccaccagggagcgcttgattacagcctggagcacagcatcaggagtcgagatcatccctccccagcgggtcactcttgctggctgaagggagttcacccactctaggatctcgttgtattcaattgtctcctccaggttctgaaggttggggttgacactgcggattgcacgcatgtatgcctttagcagctggatgtctcgcttctgctccgccagctggtgtttgtgttcagctgacgtcttctccagctctgcgatgcgtgtctgctgctgctgtaccactgagcgcaggtgcttaatgcagttatggttgggcagctcatctttgggcatctccaggccacagccctgttcacaggtcacaggccgcttcgggttgtgctcacagtcgctgaggtgagacatgaggttgtcaagccggacaacggcactacagccgaacacagcgttgtcacaggcaatctgcagctttgacaacatgttccgcatgatccgaggtactgggcgcagatgggcgaccgtcacaacactacggtccactggacatgtctgttgctgagagaaccactgggtgatgcaggcgttgcagaaagcatgttcacaatgaggtgcctgtactggctcctccaagactccactgcaaatagggcagataagatcttcgtcaacatccccctggaaacgggttacatcataccccatgtctcatcactgaaacccaggtccttccaagtgttggggggcaggttccctgttcacaaggctccaaccccctgatgcctccactcagtgccactgaagagattctcccagtaacccatcttgttggctattctccgactgagtattccttcccagtgacaagctccatcgcccaggggatgaatgtgatgtcacaatcaggagtactcactcgtcgccgcctcagacggatcctttgccccgcccaccgctgctacgcaacccggcggaagctc

SEQ ID NO: 11449 - RNA, 3943 nt, Homo sapiens
  source 1..3943: mol_type = other RNA
ctgaatagctgggactacaggtgcctgccaccacgcccggctaattttttgtatttttagtagagacggggtttcactgtgttagccaggatggtctcgaactcctgaccttgtgatccacccacctcggcctcccaaagtgctgggattacaggcgtgagccaccgcgcccggctatgaagactatttttataagtaaataattatgaaacctctgcaagtacatttccctcctcacatttacgttcttagctaggaaacactgggaggtagagacttctctgcctgcaaaggaattctagattctaaagcaaagttgcttgtgggacaaaggaaaaagatatatacatatcttctgtagaaattatcccaaaaactcaggaccactcagggaagacatggaatttaggataaaggcagaccctgggaagcacacagttcagatcactagagagctttggctgctacagaacaggagataggagggaagaatgcaggagggtacatgggaaagcagctgtgaagtgcacactactcccagacatcctcctgaaagagaagttagcactaagataagggtaggtaacaaagtaaggaagaaagggaattaaggtgagagaaaggcaaaagcagaggggaaaccttctcaagaaagggagtaatgctgaagaatttagagagttgagtaaaaggtttattattagtgcagtcaacaccatggaacagcacatacaacacaaccagcaacctgcagagacactagtgcaaagggtagggaagcctttcactgagcttcctggctccatctgagggtaaggacaggacagtatgagccttggttaaggcaggtaggggaaaggggagtggaagaaatgtagtaaccagagtaagtatagcagcgttttcaaattcctgagcacaatgtcccagagctggaaccctactcccctcaagctttccaccccaatcccagtggagccatgatccaactacccagacctgcagcaagctagcctggaataaaattctgagaggaagccattacatggtggggaggagcctttctatctccaaccacactcccacctccatattaaaataatcacacctattatctctccccttctcttactctgccagtcactctagggatcaaggtataccccaggtaacctgaaatggaactgaagtccccaggggggtgtgggtgagacacggcacagcctgtacttagagataaaatttctgatttgcatggtgaagcttagaacccagctatacagctccaaggaaacttggggaagggggagttgccttcaaaatgaatactctaaatccagagttttatgataaggccctggaagggctaggaggaaatttttccagagggcacaggcatcgatgctggactgtcatatccttcacaggaagagaggaagctcctcatttcagttggggttacagaggtttggggcagatatcgtaagttcagccgaggactcccttggctcttcctatattaaagccaaaggttgtgctgaaaaggaaaaaatataaaacacacccccatccctgtcccaccctatccagaacccccacaataggaacatcaaaagaaaagtttcaagtttgatttttttttcttttttcctttcttaaaaaaaaaaaaaggaagtaaataaattaaattgccaacaatgtggctgagatagccatgatcaggccattcttaaaaaaaagaggggggggggcagtaggtggagtttgtgaaatataaacaaacaatggccaaagaaaattatcaaagtaactaactacagtcacagggctagagaggggtctatggaacaattatggcctgtgccacaagaggcagtgccaaccatattttagcaaaagctaggagtagcttcttgctaaacacatcaacccccaacagattaacccctaccctaaaccctggcattccctaattatgaaaacttgtaggaaagaagagctcatctggaaattttcagtatcccaacctgcatactggtagacccagtgggtgcctacacctttaaggtgggctgaacagggatactgcttggcacagaggtccagtctttccctaagggccatcagtgatggccaattaacggcctcactacttatttctagagatttggctccacccttaccatttcttcaggatgtctgctgcttagagtcaacaggcctgactgctctgattccctggttttggaggagagggacgattagagattccttcctctgtcctgatcctccagggaaattgaatctctttgtgctttctgaaaataactggaaccagggaccctaagcaggaaaatggatggaggtgggggctttcccacccagactgataatttatagacattttaggggaatatggcaaagggaggaaatctgggtttcccacctgaaaggctgagcaaactaccccaaggcccttcagtgccagaagggcagggagatgtgtggctcaggtataagccacagtattaagaatggtgggtaggactcaggtcccagctgctggagtgatgggattttctgatttccatctcttcctgatagccagtcgagttctcttatatctcttccacgccatgcgcaaatatcatgacaaggcctggctcttgcaccatgtcatcccccatgtgctggttctcacaggccatcacgacaacagcctgcttgccagggatgcgcttggccacgtagttctcatagtagcgtcggttcatctgtctagtctctagtgtggccagaccctggggccagctacgctcgtgggcattttcaatcagctcgttgacaatagaagcaggacagccactctccaccagggagcgcttgattacagcctggagcacagcatcaggagtcgagatcatccctccccagcgggtcactcttgctggctgaagggagttcacccactctaggatctcgttgtattcaattgtctcctccaggttctgaaggttggggttgacactgcggattgcacgcatgtatgcctttagcagctggatgtctcgcttctgctccgccagctggtgtttgtgttcagctgacgtcttctccagctctgcgatgcgtgtctgctgctgctgtaccactgagcgcaggtgcttaatgcagttatggttgggcagctcatctttgggcatctccaggccacagccctgttcacaggtcacaggccgcttcgggttgtgctcacagtcgctgaggtgagacatgaggttgtcaagccggacaacggcactacagccgaacacagcgttgtcacaggcaatctgcagctttgacaacatgttccgcatgatccgaggtactgggcgcagatgggcgaccgtcacaacactacggtccactggacatgtctgttgctgagagaaccactgggtgatgcaggcgttgcagaaagcatgttcacaatgaggtgcctgtactggctcctccaagactccactgcaaatagggcagataagatcttcgtcaacatccccctggaaacgggttacatcataccccatgtctcatcactgaaacccaggtccttccaagtgttggggggcaggttccctgttcacaaggctccaaccccctgatgcctccactcagtgccactgaagagattctcccagtaacccatcttgttggctattctccgactgagtattccttcccagtgacaagctccatcgcccaggggatgaatgtgatgtcacaatcaggagtactcgccctggaagcggcctggagtctccgcaacctgacccagtcggagctgaggccgcagcggccacagtactgccctggtgccgggtcccagcctctcccgggaagggaagggaaaggggaaggaggggaaagaagactcctaccactcgtcgccgcctcagac

SEQ ID NO: 11450 - RNA, 3891 nt, Homo sapiens
  source 1..3891: mol_type = other RNA
ctgaatagctgggactacaggtgcctgccaccacgcccggctaattttttgtatttttagtagagacggggtttcactgtgttagccaggatggtctcgaactcctgaccttgtgatccacccacctcggcctcccaaagtgctgggattacaggcgtgagccaccgcgcccggctatgaagactatttttataagtaaataattatgaaacctctgcaagtacatttccctcctcacatttacgttcttagctaggaaacactgggaggtagagacttctctgcctgcaaaggaattctagattctaaagcaaagttgcttgtgggacaaaggaaaaagatatatacatatcttctgtagaaattatcccaaaaactcaggaccactcagggaagacatggaatttaggataaaggcagaccctgggaagcacacagttcagatcactagagagctttggctgctacagaacaggagataggagggaagaatgcaggagggtacatgggaaagcagctgtgaagtgcacactactcccagacatcctcctgaaagagaagttagcactaagataagggtaggtaacaaagtaaggaagaaagggaattaaggtgagagaaaggcaaaagcagaggggaaaccttctcaagaaagggagtaatgctgaagaatttagagagttgagtaaaaggtttattattagtgcagtcaacaccatggaacagcacatacaacacaaccagcaacctgcagagacactagtgcaaagggtagggaagcctttcactgagcttcctggctccatctgagggtaaggacaggacagtatgagccttggttaaggcaggtaggggaaaggggagtggaagaaatgtagtaaccagagtaagtatagcagcgttttcaaattcctgagcacaatgtcccagagctggaaccctactcccctcaagctttccaccccaatcccagtggagccatgatccaactacccagacctgcagcaagctagcctggaataaaattctgagaggaagccattacatggtggggaggagcctttctatctccaaccacactcccacctccatattaaaataatcacacctattatctctccccttctcttactctgccagtcactctagggatcaaggtataccccaggtaacctgaaatggaactgaagtccccaggggggtgtgggtgagacacggcacagcctgtacttagagataaaatttctgatttgcatggtgaagcttagaacccagctatacagctccaaggaaacttggggaagggggagttgccttcaaaatgaatactctaaatccagagttttatgataaggccctggaagggctaggaggaaatttttccagagggcacaggcatcgatgctggactgtcatatccttcacaggaagagaggaagctcctcatttcagttggggttacagaggtttggggcagatatcgtaagttcagccgaggactcccttggctcttcctatattaaagccaaaggttgtgctgaaaaggaaaaaatataaaacacacccccatccctgtcccaccctatccagaacccccacaataggaacatcaaaagaaaagtttcaagtttgatttttttttcttttttcctttcttaaaaaaaaaaaaaggaagtaaataaattaaattgccaacaatgtggctgagatagccatgatcaggccattcttaaaaaaaagaggggggggggcagtaggtggagtttgtgaaatataaacaaacaatggccaaagaaaattatcaaagtaactaactacagtcacagggctagagaggggtctatggaacaattatggcctgtgccacaagaggcagtgccaaccatattttagcaaaagctaggagtagcttcttgctaaacacatcaacccccaacagattaacccctaccctaaaccctggcattccctaattatgaaaacttgtaggaaagaagagctcatctggaaattttcagtatcccaacctgcatactggtagacccagtgggtgcctacacctttaaggtgggctgaacagggatactgcttggcacagaggtccagtctttccctaagggccatcagtgatggccaattaacggcctcactacttatttctagagatttggctccacccttaccatttcttcaggatgtctgctgcttagagtcaacaggcctgactgctctgattccctggttttggaggagagggacgattagagattccttcctctgtcctgatcctccagggaaattgaatctctttgtgctttctgaaaataactggaaccagggaccctaagcaggaaaatggatggaggtgggggctttcccacccagactgataatttatagacattttaggggaatatggcaaagggaggaaatctgggtttcccacctgaaaggctgagcaaactaccccaaggcccttcagtgccagaagggcagggagatgtgtggctcaggtataagccacagtattaagaatggtgggtaggactcaggtcccagctgctggagtgatgggattttctgatttccatctcttcctgatagccagtcgagttctcttatatctcttccacgccatgcgcaaatatcatgacaaggcctggctcttgcaccatgtcatcccccatgtgctggttctcacaggccatcacgacaacagcctgcttgccagggatgcgcttggccacgtagttctcatagtagcgtcggttcatctgtctagtctctagtgtggccagaccctggggccagctacgctcgtgggcattttcaatcagctcgttgacaatagaagcaggacagccactctccaccagggagcgcttgattacagcctggagcacagcatcaggagtcgagatcatccctccccagcgggtcactcttgctggctgaagggagttcacccactctaggatctcgttgtattcaattgtctcctccaggttctgaaggttggggttgacactgcggattgcacgcatgtatgcctttagcagctggatgtctcgcttctgctccgccagctggtgtttgtgttcagctgacgtcttctccagctctgcgatgcgtgtctgctgctgctgtaccactgagcgcaggtgcttaatgcagttatggttgggcagctcatctttgggcatctccaggccacagccctgttcacaggtcacaggccgcttcgggttgtgctcacagtcgctgaggtgagacatgaggttgtcaagccggacaacggcactacagccgaacacagcgttgtcacaggcaatctgcagctttgacaacatgttccgcatgatccgaggtactgggcgcagatgggcgaccgtcacaacactacggtccactggacatgtctgttgctgagagaaccactgggtgatgcaggcgttgcagaaagcatgttcacaatgaggtgcctgtactggctcctccaagactccactgcaaatagggcagataagatcttcgtcaacatccccctggaaacgggttacatcataccccatgtctcatcactgaaacccaggtccttccaagtgttggggggcaggttccctgttcacaaggctccaaccccctgatgcctccactcagtgccactgaagagattctcccagtaacccatcttgttggctattctccgactgagtattccttcccagtgacaagctccatcgcccaggggatgaatgtgatgtcacaatcaggagtactctcccgactcctcgccagtgctgctcccttctcacatttttatctctaccaccatccctcctcctgaaccccagttatttcaaccccccgccccaatacccctgggacatc

SEQ ID NO: 11451 - RNA, 3447 nt, Homo sapiens
  source 1..3447: mol_type = other RNA
ctgaatagctgggactacaggtgcctgccaccacgcccggctaattttttttgcatttttagtagagacgggtttcaccgtgttagccaggatggtctcgatctcctgacctcgtgatccacccgcctcagcctcccaaagtgctgggattacaggcgtgagccaccgcgcctggcctgctcttttaaataaacatttgccttgcaactttctattttgtttaaaatgctaccattttttcgtaagataagagatatgtttcaacctaatttccaaattactttgtgaattccatgaagattttctatacttgatacttaggaggttaaaaaatgcttttaaagtctcattaagtcttaagtaaatggaaattatagaataattttcctagatttcaatgtcaattctattttcttctgttatttctaagcagactgacatgattgattcttaaaagaaaacctgatttgagcaatctattgagcaaaacatttgtaaataaatagtgcccaattaaatcagacttattttaaaaaatatatgtcctgtactgcattgttttcattaagttataaccacaagaaatagtaacccaaatgttcaaacttctttagctgacaggccttgtttgtgtgaaacatatttattacacatacatcacactctatgcatgatctactttgctcttgagggcaggtctctgtcttattccactctgtacactcagcacctattggagtggccacagcgcataatgggtgcttccatatcagaactgacatttcagaacaactactagatgtgtttacacccagtggatgggcatccagaagtccatgccttctttcgttgtttttaagatgggtagagaagtctttcatggtcattacctcctaggatatcacattctgctttgccagtttctcataaacatgatcagttcacagccaatcccaggaggatggagcaaatgtagtggccccagtctcactgctgtgaggctcagcaggaaggtttctggccaatctgtgtctgacatggccctggcatgtgtctgctgcctggagtcctccatcgggggcggacacatgcagctctcaggaatagcctactctgaaagccagcctacattcactagaggacttatgctcagttttggcttatgtgtacagtgtgtaaaatgtaaaaaatactacccatatcaaaacagaggcttttcatctgtttccataattttaggaattcaaacttggatatgtttaaaattgaaaacactagaacttctacgcacagatagtactaagtcttacctcttaataacttaaaccttgccgtcaaacaatttcaaaatacacttatttgcaaaagtggtacaagcccaaactatggagtctctcactgttgatgaacaccatgaaatgttcagggctaaactctaccaacctagactttgcatattaaatcagggaatcagagattattttcataattgctggggtgcggggaaagagtgttttaaagtgcctattctatactgcactgcaaataatatatgtgtgtgcatacatctacatatacacacatgtaagtatgtatatgtcacctagctatatccagaagtgacattcatttattactgtagcattggcaatattcccttggaataacaccgtcatctcgtcctgttatctttctggtaattgacaaaaatacatgcttgacagctcccataaaaagcaggtatgcaagtcgtacatctgttgttttaggaggtgaatcaataaagtttgggtggggactaatagaatcctcaggttattcacttttataaacttttctttttaacctcccagcagtcccttttcctaagttaacagctttttgtatatgctgttattcaggttactagagcaggtatccattttacttgccatcaactgcccactgctgttataactgctgggatcggaactttctttgcagcataagatactgtagacgtacctctggcactcagaggaagcgtaatagtaaattagggggtcgatgcagcagcttatgctgctgacacagacacagaggaggtaggcaaagtaggcagcctctgtggtggaagtgtgagaaaggaatgagtaatgcgcaatcaggaggacgtttgtgggtccgaagcaaatgatgaagatgcagaaaacagcagctgacaggaacaaagcccgggacttcttgctgcggttggcaactgcggaagagctaagacatcgaatgatagacacataacagaccgtggaaatgatcagcggcacaaaaaagaagacagcagagaaggctgagaagtagtaggcatagtagccttcgagcagggtttcattgagcacatcatgacaggtagtgatgttgagcccgggcacctggatggtttgctccttgaggagcagaggcactacccctgcgatggccaaagcccagatggccagacaagtgaaggaagcccttcccagagtacgccaggagagggactgcatgggatacaccacagccagaaaccggtcaatgcttatgactgtcatgagcaagatagaggcgtacatgttacagtaaaatgctgcagtgacgaagcgacacaattcagacccaaactgccaatcactgccggaaaagtaatagctgatcttaaaggggagcacagacacaaacagcacatctgccgtggccaggtgcagcatgtacaccaccgccggcttcttgaccttcattttcaggatgaacacaacgatggccatgatgtttagtgggaggctgactacaaacactccggtgtacacagatgggacaaagagtgtcagccaggagctggtcaaatatccggaggcatcttctgagatgaatgcaggaagttgtttttgaagaggactgcttttattgatggagactaatctgtattcagttaacccactttcatttttctcctcatcctcccaaaatggttcatatttatcattggggttcctgagaagaaatgaccggggatctaaggtggcatttgttgcttttgattctataatcccagctcctcgggaggctgaggcaggagaattgcttgaacgcaggaggcggaggttgcagtgagctgagattgcgccattgcactccagcctggccgacagagcgagaccccatctggcctgcgggcccgggtgcgggcagacaacagcgggccgcacagactgaagcaggcggccaccagcagcagccgccgcggccccattgtcccgggctctgcgcggcgctgctccgggaggctgccccgcctcgggctgctccgcttcaccctctctcctgacttctgcgggtcggggagccggtcttcgcggcaggcagagcgcagggtgcccacgggtaagatcagggtccaagcgaccctcggcgagcgctgtgtctggggcggtt

SEQ ID NO: 11452 - RNA, 3325 nt, Homo sapiens
  source 1..3325: mol_type = other RNA
ctgaatagctgggactacaggtgcctgccaccacgcccggctaattttttttgcatttttagtagagacgggtttcaccgtgttagccaggatggtctcgatctcctgacctcgtgatccacccgcctcagcctcccaaagtgctgggattacaggcgtgagccaccgcgcctggcctgctcttttaaataaacatttgccttgcaactttctattttgtttaaaatgctaccattttttcgtaagataagagatatgtttcaacctaatttccaaattactttgtgaattccatgaagattttctatacttgatacttaggaggttaaaaaatgcttttaaagtctcattaagtcttaagtaaatggaaattatagaataattttcctagatttcaatgtcaattctattttcttctgttatttctaagcagactgacatgattgattcttaaaagaaaacctgatttgagcaatctattgagcaaaacatttgtaaataaatagtgcccaattaaatcagacttattttaaaaaatatatgtcctgtactgcattgttttcattaagttataaccacaagaaatagtaacccaaatgttcaaacttctttagctgacaggccttgtttgtgtgaaacatatttattacacatacatcacactctatgcatgatctactttgctcttgagggcaggtctctgtcttattccactctgtacactcagcacctattggagtggccacagcgcataatgggtgcttccatatcagaactgacatttcagaacaactactagatgtgtttacacccagtggatgggcatccagaagtccatgccttctttcgttgtttttaagatgggtagagaagtctttcatggtcattacctcctaggatatcacattctgctttgccagtttctcataaacatgatcagttcacagccaatcccaggaggatggagcaaatgtagtggccccagtctcactgctgtgaggctcagcaggaaggtttctggccaatctgtgtctgacatggccctggcatgtgtctgctgcctggagtcctccatcgggggcggacacatgcagctctcaggaatagcctactctgaaagccagcctacattcactagaggacttatgctcagttttggcttatgtgtacagtgtgtaaaatgtaaaaaatactacccatatcaaaacagaggcttttcatctgtttccataattttaggaattcaaacttggatatgtttaaaattgaaaacactagaacttctacgcacagatagtactaagtcttacctcttaataacttaaaccttgccgtcaaacaatttcaaaatacacttatttgcaaaagtggtacaagcccaaactatggagtctctcactgttgatgaacaccatgaaatgttcagggctaaactctaccaacctagactttgcatattaaatcagggaatcagagattattttcataattgctggggtgcggggaaagagtgttttaaagtgcctattctatactgcactgcaaataatatatgtgtgtgcatacatctacatatacacacatgtaagtatgtatatgtcacctagctatatccagaagtgacattcatttattactgtagcattggcaatattcccttggaataacaccgtcatctcgtcctgttatctttctggtaattgacaaaaatacatgcttgacagctcccataaaaagcaggtatgcaagtcgtacatctgttgttttaggaggtgaatcaataaagtttgggtggggactaatagaatcctcaggttattcacttttataaacttttctttttaacctcccagcagtcccttttcctaagttaacagctttttgtatatgctgttattcaggttactagagcaggtatccattttacttgccatcaactgcccactgctgttataactgctgggatcggaactttctttgcagcataagatactgtagacgtacctctggcactcagaggaagcgtaatagtaaattagggggtcgatgcagcagcttatgctgctgacacagacacagaggaggtaggcaaagtaggcagcctctgtggtggaagtgtgagaaaggaatgagtaatgcgcaatcaggaggacgtttgtgggtccgaagcaaatgatgaagatgcagaaaacagcagctgacaggaacaaagcccgggacttcttgctgcggttggcaactgcggaagagctaagacatcgaatgatagacacataacagaccgtggaaatgatcagcggcacaaaaaagaagacagcagagaaggctgagaagtagtaggcatagtagccttcgagcagggtttcattgagcacatcatgacaggtagtgatgttgagcccgggcacctggatggtttgctccttgaggagcagaggcactacccctgcgatggccaaagcccagatggccagacaagtgaaggaagcccttcccagagtacgccaggagagggactgcatgggatacaccacagccagaaaccggtcaatgcttatgactgtcatgagcaagatagaggcgtacatgttacagtaaaatgctgcagtgacgaagcgacacaattcagacccaaactgccaatcactgccggaaaagtaatagctgatcttaaaggggagcacagacacaaacagcacatctgccgtggccaggtgcagcatgtacaccaccgccggcttcttgaccttcattttcaggatgaacacaacgatggccatgatgtttagtgggaggctgactacaaacactccggtgtacacagatgggacaaagagtgtcagccaggagctggtcaaatatccggaggcatcttctgagatgaatgcaggaagttgtttttgaagaggactgcttttattgatggagactaatctgtattcagttaacccactttcatttttctcctcatcctcccaaaatggttcatatttatcattggggttcctgagaagaaatgaccggggatctaaggtggcatttgttgcttttgattctggcctgcgggcccgggtgcgggcagacaacagcgggccgcacagactgaagcaggcggccaccagcagcagccgccgcggccccattgtcccgggctctgcgcggcgctgctccgggaggctgccccgcctcgggctgctccgcttcaccctctctcctgacttctgcgggtcggggagccggtcttcgcggcaggcagagcgcagggtgcccacgggtaagatcagggtccaagcgaccctcggcgagcgctgtgtctggggcggtt

SEQ ID NO: 11453 - RNA, 2458 nt, Homo sapiens
  source 1..2458: mol_type = other RNA
ctgaatagctgggactacaggtgcctgccaccacgcctggctaattttttgtatttttagtagagacagggtttcactgtgttagccaggatggtctcgatctcctgacctcgtgatctgcccgtctcggcctcccaaagtgctgggattacaggctttagccactgcacccggcccatttctcttttatgaaactattctcctcaactttcctggaaaaatattgatacctgataatttgttcaaccaatcaattcaactcctacatggtctcattctgagaataccccccttctcaaaaacaatgccttctttgggtgctctgaggggtggagaccataaaatatttcctaatcagtcacatgtcaaatgatagcgttataacaagatcctattgtacgtgtatgagaccatttggttatttatggaagactctgggaattacagaacatttcaaaaatttttagcatttgctataatatggacctaaaaattttaatccccaaagcatggtgaaattctgctaatgctctgctctgaatggcgtccttagaagtggcagttattcaaagatgtcagtgagtaatccatcttctctaaacgttagtcccttttgtcctggtttctggcaagtgcttcacatgggcactgccagtattaaaaggagaagactcaaacaccagtgcatttgatgggtattgattatagacttcagctgtgggctccgtcagactacttctagatgtctctattatagaatgcctcattgtatcattcgtttcaatcatttcaaaatccatttcattccatttttctgcatcctcctcttcattctcttcctcatattcatttagcccggagctagagagcagagctttctggtcctcactctttctgtcttcttttcgctggcgatcaagaggtgaagtggctaatttatatagcacaggaaataaaataccagtagctattgatgctcccaaagaggtatacagaactacaggcaaatcagggtattttccttgaagaattccaatgactgcaggaatagccatttctcccagggaagcaccaattacaaaaaatgctgcagatttcccatggatggtcgtgtactgctcaatccaagaaacaccactcggaaatgtggttgccattgaagccccatacactgaagttgctatccagagacaaattgggttcttgtcaaaaagcaccagaaataaagatgaagtcaggctgccaatgttgctcaacacaatcatggttccaggctgtaaacaggtagcaaaaaagattgccaggcccctgcaggctgcaaatgtcccccagaagatggagttcaacccagcagcttcactttctttcatgccagcatgggtggttgcaaatgagaaaacataagagccatatgttacctcagctccaacataaaaaaagaagaacagaaaaaggagacaaagaagggcgttgtgatattttgctcttcgaaatgtctcagcagatgctcttgctttttcttgctttgagctattctttaaaaacagacaaaaaaaaatgacagaaactaagaacatgtaagtaccgataacagcataagcccacagtaaattcttatcattaggtactccaaacagagcttctgagtcagcatcagatgattggttgagtgcaggatggaagtcagactctgtgtggttttcagcagacgctgtcggacccaaagccagtttagctagcagtggagccaaaaaggcacccaaggcaaaagagaagtgtaaggcctgcatatgtggggctcctttgtccccccaaatagccaagataaggacgttaccacccaaaagtaaaaaataattcatgacatcgacaagaaatccaccaatcacagagccactcaaatatcccaaggcacgacccacaaaaatgaaagacagactactgatatttcggttcacgtttgttgccaaatcttgaaacgtgggtcccactatagcaacactcaatcccagccccaggaaggaggcacacagcatcaaggtggtgaaccaccgcagcttgctcccggtcccaccgctctgccaggagaccaccaccacctccggctccggctcattctccgccggggcctccgcctgcaggagccgctgccccgcagccgggggcccggccccacggagctccacctctaactccagctcggcggctccggagaagtcgtcttgctgccgccgcgcttctcagcagaacttctggagctccgagaagagcactggccccgaccccaggcacgggtgtccctccgggcgccacctcccagcggaccgcccggaaccggggcagagaagaggaacttcggcacgccgcaggtgttcgtggcaaaagacgctcgctctccagcaagcaggcgcatgcgcgggtcacgtggcggaaatgtggcctctcgccaaccgctatc

SEQ ID NO: 11454 - RNA, 2515 nt, Homo sapiens
  source 1..2515: mol_type = other RNA
ctgaatagctgggactacaggtgcctgccaccacgcctggctaattttttgtatttttagtagagacagggtttcactgtgttagccaggatggtctcgatctcctgacctcgtgatctgcccgtctcggcctcccaaagtgctgggattacaggctttagccactgcacccggcccatttctcttttatgaaactattctcctcaactttcctggaaaaatattgatacctgataatttgttcaaccaatcaattcaactcctacatggtctcattctgagaataccccccttctcaaaaacaatgccttctttgggtgctctgaggggtggagaccataaaatatttcctaatcagtcacatgtcaaatgatagcgttataacaagatcctattgtacgtgtatgagaccatttggttatttatggaagactctgggaattacagaacatttcaaaaatttttagcatttgctataatatggacctaaaaattttaatccccaaagcatggtgaaattctgctaatgctctgctctgaatggcgtccttagaagtggcagttattcaaagatgtcagtgagtaatccatcttctctaaacgttagtcccttttgtcctggtttctggcaagtgcttcacatgggcactgccagtattaaaaggagaagactcaaacaccagtgcatttgatgggtattgattatagacttcagctgtgggctccgtcagactacttctagatgtctctattatagaatgcctcattgtatcattcgtttcaatcatttcaaaatccatttcattccatttttctgcatcctcctcttcattctcttcctcatattcatttagcccggagctagagagcagagctttctggtcctcactctttctgtcttcttttcgctggcgatcaagaggtgaagtggctaatttatatagcacaggaaataaaataccagtagctattgatgctcccaaagaggtatacagaactacaggcaaatcagggtattttccttgaagaattccaatgactgcaggaatagccatttctcccagggaagcaccaattacaaaaaatgctgcagatttcccatggatggtcgtgtactgctcaatccaagaaacaccactcggaaatgtggttgccattgaagccccatacactgaagttgctatccagagacaaattgggttcttgtcaaaaagcaccagaaataaagatgaagtcaggctgccaatgttgctcaacacaatcatggttccaggctgtaaacaggtagcaaaaaagattgccaggcccctgcaggctgcaaatgtcccccagaagatggagttcaacccagcagcttcactttctttcatgccagcatgggtggttgcaaatgagaaaacataagagccatatgttacctcagctccaacataaaaaaagaagaacagaaaaaggagacaaagaagggcgttgtgatattttgctcttcgaaatgtctcagcagatgctcttgctttttcttgctttgagctattctttaaaaacagacaaaaaaaaatgacagaaactaagaacatgtaagtaccgataacagcataagcccacagtaaattcttatcattaggtactccaaacagagcttctgagtcagcatcagatgattggttgagtgcaggatggaagtcagactctgtgtggttttcagcagacgctgtcggacccaaagccagtttagctagcagtggagccaaaaaggcacccaaggcaaaagagaagtgtaaggcctgcatatgtggggctcctttgtccccccaaatagccaagataaggacgttaccacctgtatccagaatgccaattgaaacaccgaagatagacatcatgacagtgagtaatattgctgtcttgcaaaaaggaacaagataaagaccaacggtggtagccgacattgagattcccaaaagtaaaaaataattcatgacatcgacaagaaatccaccaatcacagagccactcaaatatcccaaggcacgacccacaaaaatgaaagacagactactgatatttcggttcacgtttgttgccaaatcttgaaacgtgggtcccactatagcaacactcaatcccagccccaggaaggaggcacacagcatcaaggtggtgaaccaccgcagcttgctcccggtcccaccgctctgccaggagaccaccaccacctccggctccggctcattctccgccggggcctccgcctgcaggagccgctgccccgcagccgggggcccggccccacggagctccacctctaactccagctcggcggctccggagaagtcgtcttgctgccgccgcgcttctcagcagaacttctggagctccgagaagagcactggccccgaccccaggcacgggtgtccctccgggcgccacctcccagcggaccgcccggaaccggggcagagaagaggaacttcggcacgccgcaggtgttcgtggcaaaagacgctcgctctcc

SEQ ID NO: 11455 - RNA, 2539 nt, Homo sapiens
  source 1..2539: mol_type = other RNA
ctgaatagctgggactacaggtgcctgccaccacgcctggctaattttttgtatttttagtagagacagggtttcactgtgttagccaggatggtctcgatctcctgacctcgtgatctgcccgtctcggcctcccaaagtgctgggattacaggctttagccactgcacccggcccatttctcttttatgaaactattctcctcaactttcctggaaaaatattgatacctgataatttgttcaaccaatcaattcaactcctacatggtctcattctgagaataccccccttctcaaaaacaatgccttctttgggtgctctgaggggtggagaccataaaatatttcctaatcagtcacatgtcaaatgatagcgttataacaagatcctattgtacgtgtatgagaccatttggttatttatggaagactctgggaattacagaacatttcaaaaatttttagcatttgctataatatggacctaaaaattttaatccccaaagcatggtgaaattctgctaatgctctgctctgaatggcgtccttagaagtggcagttattcaaagatgtcagtgagtaatccatcttctctaaacgttagtcccttttgtcctggtttctggcaagtgcttcacatgggcactgccagtattaaaaggagaagactcaaacaccagtgcatttgatgggtattgattatagacttcagctgtgggctccgtcagactacttctagatgtctctattatagaatgcctcattgtatcattcgtttcaatcatttcaaaatccatttcattccatttttctgcatcctcctcttcattctcttcctcatattcatttagcccggagctagagagcagagctttctggtcctcactctttctgtcttcttttcgctggcgatcaagaggtgaagtggctaatttatatagcacaggaaataaaataccagtagctattgatgctcccaaagaggtatacagaactacaggcaaatcagggtattttccttgaagaattccaatgactgcaggaatagccatttctcccagggaagcaccaattacaaaaaatgctgcagatttcccatggatggtcgtgtactgctcaatccaagaaacaccactcggaaatgtggttgccattgaagccccatacactgaagttgctatccagagacaaattgggttcttgtcaaaaagcaccagaaataaagatgaagtcaggctgccaatgttgctcaacacaatcatggttccaggctgtaaacaggtagcaaaaaagattgccaggcccctgcaggctgcaaatgtcccccagaagatggagttcaacccagcagcttcactttctttcatgccagcatgggtggttgcaaatgagaaaacataagagccatatgttacctcagctccaacataaaaaaagaagaacagaaaaaggagacaaagaagggcgttgtgatattttgctcttcgaaatgtctcagcagatgctcttgctttttcttgctttgagctattctttaaaaacagacaaaaaaaaatgacagaaactaagaacatgtaagtaccgataacagcataagcccacagtaaattcttatcattaggtactccaaacagagcttctgagtcagcatcagatgattggttgagtgcaggatggaagtcagactctgtgtggttttcagcagacgctgtcggacccaaagccagtttagctagcagtggagccaaaaaggcacccaaggcaaaagagaagtgtaaggcctgcatatgtggggctcctttgtccccccaaatagccaagataaggacgttaccacctgtatccagaatgccaattgaaacaccgaagatagacatcatgacagtgagtaatattgctgtcttgcaaaaaggaacaagataaagaccaacggtggtagccgacattgagattcccaaaagtaaaaaataattcatgacatcgacaagaaatccaccaatcacagagccactcaaatatcccaaggcacgacccacaaaaatgaaagacagactactgatatttcggttcacgtttgttgccaaatcttgaaacgtgggtcccactatagcaacactcaatcccagccccaggaaggaggcacacagcatcaaggtggtgaaccaccgcagcttgctcccggtcccaccgctctgccaggagaccaccaccacctccggctccggctcattctccgccggggcctccgcctgcaggagccgctgccccgcagccgggggcccggccccacggagctccacctctaactccagctcggcggctccggagaagtcgtcttgctgccgccgcgcttctcagcagaacttctggagctccgagaagagcactggccccgaccccaggcacgggtgtccctccgggcgccacctcccagcggaccgcccggaaccggggcagagaagaggaacttcggcacgccgcaggtgttcgtggcaaaagacgctcgctctccagcaagcaggcgcatgcgcgggtc

SEQ ID NO: 11456 - RNA, 8547 nt, Homo sapiens
  source 1..8547: mol_type = other RNA
ctgaatagctgggactacaggtgcctgccaccacgcttggttaatttttgtatttttagtagagacggggtttcaccatgttggccaggctggtctcaacctcctgacgtcacgtgatcagcctaccttggccttccaaagtgctgggattacaggcatgagccacccctcctggcctgggtttaactattttattttatgacagggtctcactttgttgtccaggtaccggtgcgttctctgttcactgcaacctccacctcctgagttcaagcgatcctcccacctcagcctcctgagtagctggaactacagatgcataccaccacacccggctaatttttgtatttgttgtagagacaggttttcactgtgttgcctaggctggtctcaaactcctggtgtcaagggatccactgatctcggcctcccaaagtgctgggattacagaaatgagccaccacgtctggccctgggcttacctttcaagtcaactttgattcattgtcttccttgaaacaccacattcagtgattagtcaaataatgaacattattcttgcacaactcttttgaatctatcaattactttctactcatttagtacatattcactggggagatgctctgtgccagacactgtagtaagatcaggtaattcagaggaagtatagacaccccagacctcaaacgaagacaagataaatatggacaagggaagatccacctccacattcaccattttcagtctttctgtcatttccagctaaataacgtcttcaaaaatgtttcaaaataactaagtcactatttcaaactctttcaataatagcacccttctatacactggactactcttaattttctcattataacatgatcttgcttttcttttaatttttgtctttgctttctacctgaatttttattttgcattatgaaattgataggtccattactggatggcatggttcaattctccagtatgtctgttgatttgtgttccactaaatcttccaattactcagagaggagtgttaatgactgcaactataactggatttttctatttttacttggcgtatccaattttgtttatgagttttgaagctctgtgtcctcatatacatttgggacaatattctcctgaaaaattgacaatcataattatttaggaggcctcattattcctgaaaagtttctctgctttcaaatctactttgtctgattttatatatatacaccacagctgtctttgattaatgcttgcatgaggtatcttttcccactcttttctttcaatctgctctataacttttattcttatttataagtgtattgcaggtggctttctttagtcagcatatttatttttaacacattctgatgatctctagtttttacttaatgcatttagataatttacatataatgttattatagataagtttttagatagatctactatttaataatttattaaccttttttccctttgttttaattcttctatgttcctctgtctatcttgttttggtttatttcaatctggttgttaagtggtctagggattaccatatacatatataacttttcacagtatactaagaatcaatattttaccattcaagttgaatatagaaacttcatcaagagttagtcccattacatttacccttttatcttatgtatgtagtacatctagatacaatgacaactgcatcagataaagttacaatttttgctttcaaccatcaaacataccttaaggaactcaagagaagaataatagtctgttatgtctacccagacattttctatttctgcttttgttccttcattgatgatgttctaagtttccttctggtatcacttttcttatctcaaacctttgctaattcttttccagcagttttgctaggactgagaatgtatttatttaccttccaatgagaatgcatttatttgcctttatgtctggaagatacttttgctccacataccattctgggttgataatgtatttttcctttggtatttactgaatgttatgacatttttttctggctcctgggttcccgatgagaaatctacaatcattcatttggtattttatctttcatttccctttggctgctttcaaaattgttttgtgttttcttaattttccgcagtttgattatgatatgtcttgcaatgggtttcttttggtttatcctgcttgacatttactgaactttaaaaatctggtttatatcttttgagaaatttgatacattttcagccattaattcttcacagttttatcccacaaagacctctttgtcctcttacaataatgtgaatgtttccagattacaataatgtgaatgttagatttgttattttttatttgtccctgagcctctgttcagggacaataaaatcctcctttctttctataggtcagattctgtaggtattcttgttccgttttcaagttcattgactttttccttagtcttctgcatactgctattgagatcatccaattaagctttttatttcccctaatagttttggttaatactttttttaattcttaagtttaaattggtgtttacatattccaaatatttggtgagactttccaactttccattcacttcatgaatgctatcccgtaattctaggagcattgttataataactgctttaatgtatgtgtcagatgattttgacatatgtgtcctctcaatattgttatgcaaggattctctttgccatgtgaattaagatctccctggtttttcataatgctgaatattttggggcttgtaacctggacttctttggattatgtgatgagacactgtgtcttgttgaaatcttaaggataatattgctctttttgtttttgcaggcacacaattgccttgtatttaagctccaagtaccaaccagacttccatgtgttgttgtttcacagataactctatttgaaagccttgacactgcggatgagagatctctggagtgtgtgcaaccagtggtcagtgaggactggaaagtggaccattgtttagttcagtcctcaggctctttttaggtaagttgtttgggattagacccacttattcacagctggcaggtgcgtccacaagctcatgaacaactttatgggtttgctttctacagtatctgtccaggcacattctagttacttgacacatcctggtttcagtcctctcaccagaaagccagggctgtatttacccaggtggctctgccctgcacttttcacagttgcctcacattcaagccgcatttatcgtgtcagctcccgaggtggacaacaggagtctttctgcagcgtcagtgcccatcacacttcctgctgcagaatacatcctccataaacaccatagcatggatgatgacagaggtgaatgaaaagaaagaaaaacattctggtgatgctgtgcaggaaggatctacagtatttgtcaagacattgggtggagagatttgagggagaggagacaaagacactgggaagtcttgagcctagtgtggtagacacaaaagagattctgaattaatagctgatgaatgaatccactcatttatttgtatttgttatgtgaatgaatgttacatgaatgacctggcatggagaaaacagatggtgagactatgtgctagggtaaagcaagagctcaagttttttttttttttttaatttagaaaaaaatctgcttttcatatctggttttcctatttaaaactatgtgatttgaggaaaatggtttaactcctctgagctttagtgtcatctacaaaatttggataatgatactgagggaagctgaaaagccgtatcaaccaacttatacaaaaaataataaacattcacttccatttctaatgcatggtgctgaaaaagtccttgtatgtggaatattgttcacctttaaggaacctgctctcaagagctgatgagggactttttttagtgcagttctgttgtcactggctgttgggctcatttagttggcaccaacaaatctctgtcttgctgctttttttcctcttgtggcccagtcatctagcttttcccttcttcagagatcttagtcactcttcttttccgtagtctccttaaggaactcaagggaagaataatagtctgttatgtctacccagacatgttctatttctgcttttgttccttcactgatgatgttctaagtttccttctggtatcatttttcttatctcaaatctttgctaattcttttccagcagtcttcctaagaatgagaatgtatttacttaccttccactgagaatgcatttatttgcctttatgtctggaagatacttttgctccacatagcattctgggtcgatatgtctttttcttttgttacttaccgaatgttatgacattttttctggcccctatggttcctgatgcgaaatctacaatcattcatttggtagtttctctttcatttccctttggctgctttcaaaattgttttgtattttcttagttttcagcagtttgattatgatatgccttgctatgggtttctttgggtttatcctgattgacatttactgaactttaaaaatctggtttatatcttttgacaaatttgaaccattttcagctattaattgttcaaagttttatcccacaaagaccactttgtcctcttctttccagattacaataatgtgaatgttggatttgttattttttatttgtgcctgagcctctgttcagagacaataaaatcctcctttctctctatagttcagattatgtaggtattcgtgttctgttttcaagttcattgactttttccttagtcttctgcattcgattatggagatcctccaattaagctttttatttcccctaagagttttggttaatacatttttttaattcttaagtttaaattggtgtttatgtattcgaaatatttggtgagactttccaactttccattcacttcacgaatgttatccccgattctaggagcattgttataatatctgctttaatgtatgtgtcagatgattttgacatctgtgtcctctcaatattgttattcgaggattctctttgccatgtgaattaagatctccctgttttttcataatgctgaatattgtggggcttgtaacctggacttctttggattatgtgatgagacactgtgtcttgttgaaatcttaaggataatattgctatttttgtttttgcaggcacacaattgccttgtatttaagctccaagtaccaaccagactttcatgtgttgtcgtttcaaagataactctatttgaaagccttgacactgctgttcagagatctccaaagtgtgtgcaacccagtggtcagtgaggactggaaagtgggccattgcacagttcagctctcaggctctttttaggtaagttgttcgggattagagccacttattcacagctggcaggtgcgtccacaagctcatgaacaactttatggttttgctttctacagtatctgtccaggcacattctagttacttgacacatcttggtttcagtcctctcaccagaaagctggggctgtatttaaccaggtggctctgtcctccacttttcacaattgtctcacatttaggaccaagctgcaggcagaaacagggagaaaagagcagttttatatgtcctttggtttcacagctcctcgaagaaacagaaaattaattacacagtagatctacactatactgaatgccagcaggaagctgtcaccagtcctgtattgttgctgctcctatgtcttgaaccaaagacaccgagagcagtgtcttgctctcagacactgactcgggtttgggtacctaaataataaagcttggagaatgtgggcattgatcccactacctcttgcatgctaagcaagcgctctaccacttgagctaattccccatatcagggaagctttgtttatccttagtgggtggcctggaacacaggtgatttcagggccttcagcgggaaagcagggctctactaagagcagatcttctcattgatggcgcagggcaaggtgcagtggctactcattctctgcaaagaaggaggaaaaaagggaagaaggagaaagtcacaaagggaaaactcacgctgccaaaatgtgaagtttagggtattccaggacagaaaaagacacgtcccagcaaagaagacctatctagacctgcccagctaaagtgtcactgatttttaaaaaataattaaataattaaaaatgattaaatgattgtgtgtgtattgcatgtgtgtgtgtgtgtgtttataaaagtgggatggcattatcacttgttccttgtagctgagactctctgggggttgtgagatggtccagatttctggaaggcacaaaagggattctgaattaatatctgatgaatgaatccactcatttatttgtatttgttatgtgaatgaatgttacaggaatcacctggtgtggagaaaacagatggcaagactatgtgctagggtaaagcaagagctcacgtgtttttgtttttggttttttaatttagaaaaaaaatctgcttttcatatctggttttcctatttaaagctatgtgatttaaggaaaatggtttaactcctctgagctttagtgtcatctacaaaatttggataatgatactgagggaagctgaaaagccatatcaaccaacttatacaaaaaataataaacattcacttccatttctaatgcatggtgctgaaaaagtccttgtatgtggaatattgttcacctttaaggaacctgctctcaagagctgatgcgggactttttttagggcagttctgttgtctctggctgttttgttcatttaattggcacctacaagtctctttgaacattaaaataaaataaagattgtggaggaatagaatacaaacacatagtaaggtgagatttgcataacagagtatagtaaacgatttgtgcctgattctttttgcattctctttgaatcatttttagcctttattctaagtccccaattattgtcatccttttcccaacaagattgtttctctccgccacggacattctggtcagggtctctgcttaaccatcttgacctcctgaacactctgtttgtcctgataacctgatttatgctcaaatgatgctcttccataggacggcttcctgctttgcccaaagagcattcaatttttcaagctgtttagggctccttcctcacccagggtctatttgaaaccttagagggaaggctattctttccaggaagagaaccctgctgggttgtaacctcaatctgtaaatccactggggtaactggggttagctcagttactccagagcttgctctctgagaactggatggtgctgctacttcccataaaggctgaataaaaagaggcatctgcaggcaggagaaagcgctatggtcattgctggaagattccttctgaccattagctatctctctgacctggtgtgagaagggtgacaaaaatcggagacttgaaaacaggccaaaaaaaaaaaaatggattcaaaagaattttaaaagaatcatgcacaagttcttaattagattcttttatccaaatccattttgtctggaaaataataccttactacgtatctgtattctattcctccataatctattttattttattttaatgttcacaagaagctggatgctagctaccaaatgagcaaatcagccacgataacagaactgcactaaaatctctcatcagatattgatacagtcaagaccctcatgagtgcctatgatacaaattcagtgtgagaggccagctttccgcaaggagaaggcaaccaaagcggtagctaatactgagcagttcctattgcccagatccatttctaggtgctgagatccagccagagaatcccacagtcctcatttttcatatgaagaaacatgtgagtgattcaccaccccaatcctcatgtatcatcagttttcaaacaaagccaagtagcctcctgtgcaaaaagctctcctaacccccagttgccttgataggtaaaagtattcttatgacagtgctagaaaaacacgggcacaagtgttccggcaaggtgactagaaggcaaggctaaagttgtcaaggtgacaaagtccctgatggtcctcttgaaagctgaacgtgccacctcatatgtatatgtgtatgtgtggatgcatatgtgtatgttgtgtgtacacacctacacatatatctacaaatgcatgtgtgtatgcatgcatgtgtgtacacgtgcatgcgcacatgtatctgtatacatgtattatgtacacagtatgcatgtgtacatgtatgtgtgtctgtgcatgtgtagatgtatacatgcatgtacacatgcatctacatatgcatgtgtatgcctaaatgtgtgtacaagtgcgtgcatatgtgcactatacatatgtgtacattacgtgtgtgtatgtttctacacgtgtatctgc

SEQ ID NO: 11457 - RNA, 9000 nt, Homo sapiens
  source 1..9000: mol_type = other RNA
ctgaatagctgggactacaggtgcctgccaccacgcttggttaatttttgtatttttagtagagacggggtttcaccatgttggccaggctggtctcaacctcctgacgtcacgtgatcagcctaccttggccttccaaagtgctgggattacaggcatgagccacccctcctggcctgggtttaactattttattttatgacagggtctcactttgttgtccaggtaccggtgcgttctctgttcactgcaacctccacctcctgagttcaagcgatcctcccacctcagcctcctgagtagctggaactacagatgcataccaccacacccggctaatttttgtatttgttgtagagacaggttttcactgtgttgcctaggctggtctcaaactcctggtgtcaagggatccactgatctcggcctcccaaagtgctgggattacagaaatgagccaccacgtctggccctgggcttacctttcaagtcaactttgattcattgtcttccttgaaacaccacattcagtgattagtcaaataatgaacattattcttgcacaactcttttgaatctatcaattactttctactcatttagtacatattcactggggagatgctctgtgccagacactgtagtaagatcaggtaattcagaggaagtatagacaccccagacctcaaacgaagacaagataaatatggacaagggaagatccacctccacattcaccattttcagtctttctgtcatttccagctaaataacgtcttcaaaaatgtttcaaaataactaagtcactatttcaaactctttcaataatagcacccttctatacactggactactcttaattttctcattataacatgatcttgcttttcttttaatttttgtctttgctttctacctgaatttttattttgcattatgaaattgataggtccattactggatggcatggttcaattctccagtatgtctgttgatttgtgttccactaaatcttccaattactcagagaggagtgttaatgactgcaactataactggatttttctatttttacttggcgtatccaattttgtttatgagttttgaagctctgtgtcctcatatacatttgggacaatattctcctgaaaaattgacaatcataattatttaggaggcctcattattcctgaaaagtttctctgctttcaaatctactttgtctgattttatatatatacaccacagctgtctttgattaatgcttgcatgaggtatcttttcccactcttttctttcaatctgctctataacttttattcttatttataagtgtattgcaggtggctttctttagtcagcatatttatttttaacacattctgatgatctctagtttttacttaatgcatttagataatttacatataatgttattatagataagtttttagatagatctactatttaataatttattaaccttttttccctttgttttaattcttctatgttcctctgtctatcttgttttggtttatttcaatctggttgttaagtggtctagggattaccatatacatatataacttttcacagtatactaagaatcaatattttaccattcaagttgaatatagaaacttcatcaagagttagtcccattacatttacccttttatcttatgtatgtagtacatctagatacaatgacaactgcatcagataaagttacaatttttgctttcaaccatcaaacataccttaaggaactcaagagaagaataatagtctgttatgtctacccagacattttctatttctgcttttgttccttcattgatgatgttctaagtttccttctggtatcacttttcttatctcaaacctttgctaattcttttccagcagttttgctaggactgagaatgtatttatttaccttccaatgagaatgcatttatttgcctttatgtctggaagatacttttgctccacataccattctgggttgataatgtatttttcctttggtatttactgaatgttatgacatttttttctggctcctgggttcccgatgagaaatctacaatcattcatttggtattttatctttcatttccctttggctgctttcaaaattgttttgtgttttcttaattttccgcagtttgattatgatatgtcttgcaatgggtttcttttggtttatcctgcttgacatttactgaactttaaaaatctggtttatatcttttgagaaatttgatacattttcagccattaattcttcacagttttatcccacaaagacctctttgtcctcttacaataatgtgaatgtttccagattacaataatgtgaatgttagatttgttattttttatttgtccctgagcctctgttcagggacaataaaatcctcctttctttctataggtcagattctgtaggtattcttgttccgttttcaagttcattgactttttccttagtcttctgcatactgctattgagatcatccaattaagctttttatttcccctaatagttttggttaatactttttttaattcttaagtttaaattggtgtttacatattccaaatatttggtgagactttccaactttccattcacttcatgaatgctatcccgtaattctaggagcattgttataataactgctttaatgtatgtgtcagatgattttgacatatgtgtcctctcaatattgttatgcaaggattctctttgccatgtgaattaagatctccctggtttttcataatgctgaatattttggggcttgtaacctggacttctttggattatgtgatgagacactgtgtcttgttgaaatcttaaggataatattgctctttttgtttttgcaggcacacaattgccttgtatttaagctccaagtaccaaccagacttccatgtgttgttgtttcacagataactctatttgaaagccttgacactgcggatgagagatctctggagtgtgtgcaaccagtggtcagtgaggactggaaagtggaccattgtttagttcagtcctcaggctctttttaggtaagttgtttgggattagacccacttattcacagctggcaggtgcgtccacaagctcatgaacaactttatgggtttgctttctacagtatctgtccaggcacattctagttacttgacacatcctggtttcagtcctctcaccagaaagccagggctgtatttacccaggtggctctgccctgcacttttcacagttgcctcacattcaagctacaggcagaaacagggagaaaagagcaattgtttatgtcccttggtttcacagctcctcaaagaagcagaaaattaattacacggtagatctacactatactgaatgccaggagggagccgtcaccagccctgtattgttgctgctcctacatcttgaaccaaagcagcatcctgttctctgacttgggtttggagacctgagtgtttggagacccagggtctaaataataaagtttggagaatgtgggcatcgatcccactacctcttgcatgctaagcaagcgctctaccacttgagctaattcccccacatcaggggagctttattgatccttagtgggtggcctggaacacaggggatttcagggccttcagcgggaaagcagggctctactaagagcagatcttctcactgatggcccagggcaaggtgcagtggctactcattctccgcatttatcgtgtcagctcccgaggtggacaacaggagtctttctgcagcgtcagtgcccatcacacttcctgctgcagaatacatcctccataaacaccatagcatggatgatgacagaggtgaatgaaaagaaagaaaaacattctggtgatgctgtgcaggaaggatctacagtatttgtcaagacattgggtggagagatttgagggagaggagacaaagacactgggaagtcttgagcctagtgtggtagacacaaaagagattctgaattaatagctgatgaatgaatccactcatttatttgtatttgttatgtgaatgaatgttacatgaatgacctggcatggagaaaacagatggtgagactatgtgctagggtaaagcaagagctcaagttttttttttttttttaatttagaaaaaaatctgcttttcatatctggttttcctatttaaaactatgtgatttgaggaaaatggtttaactcctctgagctttagtgtcatctacaaaatttggataatgatactgagggaagctgaaaagccgtatcaaccaacttatacaaaaaataataaacattcacttccatttctaatgcatggtgctgaaaaagtccttgtatgtggaatattgttcacctttaaggaacctgctctcaagagctgatgagggactttttttagtgcagttctgttgtcactggctgttgggctcatttagttggcaccaacaaatctctgtcttgctgctttttttcctcttgtggcccagtcatctagcttttcccttcttcagagatcttagtcactcttcttttccgtagtctccttaaggaactcaagggaagaataatagtctgttatgtctacccagacatgttctatttctgcttttgttccttcactgatgatgttctaagtttccttctggtatcatttttcttatctcaaatctttgctaattcttttccagcagtcttcctaagaatgagaatgtatttacttaccttccactgagaatgcatttatttgcctttatgtctggaagatacttttgctccacatagcattctgggtcgatatgtctttttcttttgttacttaccgaatgttatgacattttttctggcccctatggttcctgatgcgaaatctacaatcattcatttggtagtttctctttcatttccctttggctgctttcaaaattgttttgtattttcttagttttcagcagtttgattatgatatgccttgctatgggtttctttgggtttatcctgattgacatttactgaactttaaaaatctggtttatatcttttgacaaatttgaaccattttcagctattaattgttcaaagttttatcccacaaagaccactttgtcctcttctttccagattacaataatgtgaatgttggatttgttattttttatttgtgcctgagcctctgttcagagacaataaaatcctcctttctctctatagttcagattatgtaggtattcgtgttctgttttcaagttcattgactttttccttagtcttctgcattcgattatggagatcctccaattaagctttttatttcccctaagagttttggttaatacatttttttaattcttaagtttaaattggtgtttatgtattcgaaatatttggtgagactttccaactttccattcacttcacgaatgttatccccgattctaggagcattgttataatatctgctttaatgtatgtgtcagatgattttgacatctgtgtcctctcaatattgttattcgaggattctctttgccatgtgaattaagatctccctgttttttcataatgctgaatattgtggggcttgtaacctggacttctttggattatgtgatgagacactgtgtcttgttgaaatcttaaggataatattgctatttttgtttttgcaggcacacaattgccttgtatttaagctccaagtaccaaccagactttcatgtgttgtcgtttcaaagataactctatttgaaagccttgacactgctgttcagagatctccaaagtgtgtgcaacccagtggtcagtgaggactggaaagtgggccattgcacagttcagctctcaggctctttttaggtaagttgttcgggattagagccacttattcacagctggcaggtgcgtccacaagctcatgaacaactttatggttttgctttctacagtatctgtccaggcacattctagttacttgacacatcttggtttcagtcctctcaccagaaagctggggctgtatttaaccaggtggctctgtcctccacttttcacaattgtctcacatttaggaccaagctgcaggcagaaacagggagaaaagagcagttttatatgtcctttggtttcacagctcctcgaagaaacagaaaattaattacacagtagatctacactatactgaatgccagcaggaagctgtcaccagtcctgtattgttgctgctcctatgtcttgaaccaaagacaccgagagcagtgtcttgctctcagacactgactcgggtttgggtacctaaataataaagcttggagaatgtgggcattgatcccactacctcttgcatgctaagcaagcgctctaccacttgagctaattccccatatcagggaagctttgtttatccttagtgggtggcctggaacacaggtgatttcagggccttcagcgggaaagcagggctctactaagagcagatcttctcattgatggcgcagggcaaggtgcagtggctactcattctctgcaaagaaggaggaaaaaagggaagaaggagaaagtcacaaagggaaaactcacgctgccaaaatgtgaagtttagggtattccaggacagaaaaagacacgtcccagcaaagaagacctatctagacctgcccagctaaagtgtcactgatttttaaaaaataattaaataattaaaaatgattaaatgattgtgtgtgtattgcatgtgtgtgtgtgtgtgtttataaaagtgggatggcattatcacttgttccttgtagctgagactctctgggggttgtgagatggtccagatttctggaaggcacaaaagggattctgaattaatatctgatgaatgaatccactcatttatttgtatttgttatgtgaatgaatgttacaggaatcacctggtgtggagaaaacagatggcaagactatgtgctagggtaaagcaagagctcacgtgtttttgtttttggttttttaatttagaaaaaaaatctgcttttcatatctggttttcctatttaaagctatgtgatttaaggaaaatggtttaactcctctgagctttagtgtcatctacaaaatttggataatgatactgagggaagctgaaaagccatatcaaccaacttatacaaaaaataataaacattcacttccatttctaatgcatggtgctgaaaaagtccttgtatgtggaatattgttcacctttaaggaacctgctctcaagagctgatgcgggactttttttagggcagttctgttgtctctggctgttttgttcatttaattggcacctacaagtctctttgaacattaaaataaaataaagattgtggaggaatagaatacaaacacatagtaaggtgagatttgcataacagagtatagtaaacgatttgtgcctgattctttttgcattctctttgaatcatttttagcctttattctaagtccccaattattgtcatccttttcccaacaagattgtttctctccgccacggacattctggtcagggtctctgcttaaccatcttgacctcctgaacactctgtttgtcctgataacctgatttatgctcaaatgatgctcttccataggacggcttcctgctttgcccaaagagcattcaatttttcaagctgtttagggctccttcctcacccagggtctatttgaaaccttagagggaaggctattctttccaggaagagaaccctgctgggttgtaacctcaatctgtaaatccactggggtaactggggttagctcagttactccagagcttgctctctgagaactggatggtgctgctacttcccataaaggctgaataaaaagaggcatctgcaggcaggagaaagcgctatggtcattgctggaagattccttctgaccattagctatctctctgacctggtgtgagaagggtgacaaaaatcggagacttgaaaacaggccaaaaaaaaaaaaatggattcaaaagaattttaaaagaatcatgcacaagttcttaattagattcttttatccaaatccattttgtctggaaaataataccttactacgtatctgtattctattcctccataatctattttattttattttaatgttcacaagaagctggatgctagctaccaaatgagcaaatcagccacgataacagaactgcactaaaatctctcatcagatattgatacagtcaagaccctcatgagtgcctatgatacaaattcagtgtgagaggccagctttccgcaaggagaaggcaaccaaagcggtagctaatactgagcagttcctattgcccagatccatttctaggtgctgagatccagccagagaatcccacagtcctcatttttcatatgaagaaacatgtgagtgattcaccaccccaatcctcatgtatcatcagttttcaaacaaagccaagtagcctcctgtgcaaaaagctctcctaacccccagttgccttgataggtaaaagtattcttatgacagtgctagaaaaacacgggcacaagtgttccggcaaggtgactagaaggcaaggctaaagttgtcaaggtgacaaagtccctgatggtcctcttgaaagctgaacgtgccacctcatatgtatatgtgtatgtgtggatgcatatgtgtatgttgtgtgtacacacctacacatatatctacaaatgcatgtgtgtatgcatgcatgtgtgtacacgtgcatgcgcacatgtatctgtatacatgtattatgtacacagtatgcatgtgtacatgtatgtgtgtctgtgcatgtgtagatgtatacatgcatgtacacatgcatctacatatgcatgtgtatgcctaaatgtgtgtacaagtgcgtgcatatgtgcactatacatatgtgtacattacgtgtgtgtatgtttctacacgtgtatctgc

SEQ ID NO: 11458 - RNA, 9669 nt, Homo sapiens
  source 1..9669: mol_type = other RNA
ctgaatagctgggactacaggtgcctgccaccacgcttggttaatttttgtatttttagtagagacggggtttcaccatgttggccaggctggtctcaacctcctgacgtcacgtgatcagcctaccttggccttccaaagtgctgggattacaggcatgagccacccctcctggcctgggtttaactattttattttatgacagggtctcactttgttgtccaggtaccggtgcgttctctgttcactgcaacctccacctcctgagttcaagcgatcctcccacctcagcctcctgagtagctggaactacagatgcataccaccacacccggctaatttttgtatttgttgtagagacaggttttcactgtgttgcctaggctggtctcaaactcctggtgtcaagggatccactgatctcggcctcccaaagtgctgggattacagaaatgagccaccacgtctggccctgggcttacctttcaagtcaactttgattcattgtcttccttgaaacaccacattcagtgattagtcaaataatgaacattattcttgcacaactcttttgaatctatcaattactttctactcatttagtacatattcactggggagatgctctgtgccagacactgtagtaagatcaggtaattcagaggaagtatagacaccccagacctcaaacgaagacaagataaatatggacaagggaagatccacctccacattcaccattttcagtctttctgtcatttccagctaaataacgtcttcaaaaatgtttcaaaataactaagtcactatttcaaactctttcaataatagcacccttctatacactggactactcttaattttctcattataacatgatcttgcttttcttttaatttttgtctttgctttctacctgaatttttattttgcattatgaaattgataggtccattactggatggcatggttcaattctccagtatgtctgttgatttgtgttccactaaatcttccaattactcagagaggagtgttaatgactgcaactataactggatttttctatttttacttggcgtatccaattttgtttatgagttttgaagctctgtgtcctcatatacatttgggacaatattctcctgaaaaattgacaatcataattatttaggaggcctcattattcctgaaaagtttctctgctttcaaatctactttgtctgattttatatatatacaccacagctgtctttgattaatgcttgcatgaggtatcttttcccactcttttctttcaatctgctctataacttttattcttatttataagtgtattgcaggtggctttctttagtcagcatatttatttttaacacattctgatgatctctagtttttacttaatgcatttagataatttacatataatgttattatagataagtttttagatagatctactatttaataatttattaaccttttttccctttgttttaattcttctatgttcctctgtctatcttgttttggtttatttcaatctggttgttaagtggtctagggattaccatatacatatataacttttcacagtatactaagaatcaatattttaccattcaagttgaatatagaaacttcatcaagagttagtcccattacatttacccttttatcttatgtatgtagtacatctagatacaatgacaactgcatcagataaagttacaatttttgctttcaaccatcaaacataccttaaggaactcaagagaagaataatagtctgttatgtctacccagacattttctatttctgcttttgttccttcattgatgatgttctaagtttccttctggtatcacttttcttatctcaaacctttgctaattcttttccagcagttttgctaggactgagaatgtatttatttaccttccaatgagaatgcatttatttgcctttatgtctggaagatacttttgctccacataccattctgggttgataatgtatttttcctttggtatttactgaatgttatgacatttttttctggctcctgggttcccgatgagaaatctacaatcattcatttggtattttatctttcatttccctttggctgctttcaaaattgttttgtgttttcttaattttccgcagtttgattatgatatgtcttgcaatgggtttcttttggtttatcctgcttgacatttactgaactttaaaaatctggtttatatcttttgagaaatttgatacattttcagccattaattcttcacagttttatcccacaaagacctctttgtcctcttacaataatgtgaatgtttccagattacaataatgtgaatgttagatttgttattttttatttgtccctgagcctctgttcagggacaataaaatcctcctttctttctataggtcagattctgtaggtattcttgttccgttttcaagttcattgactttttccttagtcttctgcatactgctattgagatcatccaattaagctttttatttcccctaatagttttggttaatactttttttaattcttaagtttaaattggtgtttacatattccaaatatttggtgagactttccaactttccattcacttcatgaatgctatcccgtaattctaggagcattgttataataactgctttaatgtatgtgtcagatgattttgacatatgtgtcctctcaatattgttatgcaaggattctctttgccatgtgaattaagatctccctggtttttcataatgctgaatattttggggcttgtaacctggacttctttggattatgtgatgagacactgtgtcttgttgaaatcttaaggataatattgctctttttgtttttgcaggcacacaattgccttgtatttaagctccaagtaccaaccagacttccatgtgttgttgtttcacagataactctatttgaaagccttgacactgcggatgagagatctctggagtgtgtgcaaccagtggtcagtgaggactggaaagtggaccattgtttagttcagtcctcaggctctttttaggtaagttgtttgggattagacccacttattcacagctggcaggtgcgtccacaagctcatgaacaactttatgggtttgctttctacagtatctgtccaggcacattctagttacttgacacatcctggtttcagtcctctcaccagaaagccagggctgtatttacccaggtggctctgccctgcacttttcacagttgcctcacattcaagctacaggcagaaacagggagaaaagagcaattgtttatgtcccttggtttcacagctcctcaaagaagcagaaaattaattacacggtagatctacactatactgaatgccaggagggagccgtcaccagccctgtattgttgctgctcctacatcttgaaccaaagcagcatcctgttctctgacttgggtttggagacctgagtgtttggagacccagggtctaaataataaagtttggagaatgtgggcatcgatcccactacctcttgcatgctaagcaagcgctctaccacttgagctaattcccccacatcaggggagctttattgatccttagtgggtggcctggaacacaggggatttcagggccttcagcgggaaagcagggctctactaagagcagatcttctcactgatggcccagggcaaggtgcagtggctactcattctctgcaaagaaggaagaggaaagggaacaaggagaaagtcaaaaagggaaaactcacactgccaaaatgtcaagtttagggtattccgggacagaaaaaggcacattccaggaaaggaggccctgcctagacctgcccatctaaagtgtcactgatttttaaaaaatgattaaataattaaaaatgattaaatgattttgtgtgtgtgtgttgtgtgtgtgtgtttataaaagtgagatagtattatcacttgttccttgtagctgagactctctggggattttgagatggtacagatttctggaaggcaaaaagctcctgttgttttcataactaggccctttcaggaatgaagccagcgtgctgaccactaccttaggaaacccctggggagtgcttctttcacttgcatctgagatataggttgcctccttgctaaggtgtgtcatgtacaagttacatgtccaactatatctcagaacaacaacaacaaaattacagagcagagccataaagaataagagacaagatcatatcagagtgtaagaatatgtaaaatattagagtgtaagaatcaaaattcagctatgcagagaaggagtggacatatggtggagaaaaccgggctgttcgtaggaattcctgtgtgaagaaataaacctgttcaatttaagtgctgtgtgtgtgtgtgtgtgtgtgtgtgtgtgtgaaatacacacggagggaagcagtgattgaaaagcctggccacttggagatatgttggtagagttttatgaaaactcccaagagtaattgaaaaaatcccaggcagaatgcttaaataattaaagcaacatgttagagaaaggtgtttagttttgaatgtcagagcttgaacatgagaaaatagaaattgaagagaaagagaaagaagtcataaagatattaaaggattgagatttacccgcatttatcgtgtcagctcccgaggtggacaacaggagtctttctgcagcgtcagtgcccatcacacttcctgctgcagaatacatcctccataaacaccatagcatggatgatgacagaggtgaatgaaaagaaagaaaaacattctggtgatgctgtgcaggaaggatctacagtatttgtcaagacattgggtggagagatttgagggagaggagacaaagacactgggaagtcttgagcctagtgtggtagacacaaaagagattctgaattaatagctgatgaatgaatccactcatttatttgtatttgttatgtgaatgaatgttacatgaatgacctggcatggagaaaacagatggtgagactatgtgctagggtaaagcaagagctcaagttttttttttttttttaatttagaaaaaaatctgcttttcatatctggttttcctatttaaaactatgtgatttgaggaaaatggtttaactcctctgagctttagtgtcatctacaaaatttggataatgatactgagggaagctgaaaagccgtatcaaccaacttatacaaaaaataataaacattcacttccatttctaatgcatggtgctgaaaaagtccttgtatgtggaatattgttcacctttaaggaacctgctctcaagagctgatgagggactttttttagtgcagttctgttgtcactggctgttgggctcatttagttggcaccaacaaatctctgtcttgctgctttttttcctcttgtggcccagtcatctagcttttcccttcttcagagatcttagtcactcttcttttccgtagtctccgaatgttatgacattttttctggcccctatggttcctgatgcgaaatctacaatcattcatttggtagtttctctttcatttccctttggctgctttcaaaattgttttgtattttcttagttttcagcagtttgattatgatatgccttgctatgggtttctttgggtttatcctgattgacatttactgaactttaaaaatctggtttatatcttttgacaaatttgaaccattttcagctattaattgttcaaagttttatcccacaaagaccactttgtcctcttctttccagattacaataatgtgaatgttggatttgttattttttatttgtgcctgagcctctgttcagagacaataaaatcctcctttctctctatagttcagattatgtaggtattcgtgttctgttttcaagttcattgactttttccttagtcttctgcattcgattatggagatcctccaattaagctttttatttcccctaagagttttggttaatacatttttttaattcttaagtttaaattggtgtttatgtattcgaaatatttggtgagactttccaactttccattcacttcacgaatgttatccccgattctaggagcattgttataatatctgctttaatgtatgtgtcagatgattttgacatctgtgtcctctcaatattgttattcgaggattctctttgccatgtgaattaagatctccctgttttttcataatgctgaatattgtggggcttgtaacctggacttctttggattatgtgatgagacactgtgtcttgttgaaatcttaaggataatattgctatttttgtttttgcaggcacacaattgccttgtatttaagctccaagtaccaaccagactttcatgtgttgtcgtttcaaagataactctatttgaaagccttgacactgctgttcagagatctccaaagtgtgtgcaacccagtggtcagtgaggactggaaagtgggccattgcacagttcagctctcaggctctttttaggtaagttgttcgggattagagccacttattcacagctggcaggtgcgtccacaagctcatgaacaactttatggttttgctttctacagtatctgtccaggcacattctagttacttgacacatcttggtttcagtcctctcaccagaaagctggggctgtatttaaccaggtggctctgtcctccacttttcacaattgtctcacatttaggaccaagctgcaggcagaaacagggagaaaagagcagttttatatgtcctttggtttcacagctcctcgaagaaacagaaaattaattacacagtagatctacactatactgaatgccagcaggaagctgtcaccagtcctgtattgttgctgctcctatgtcttgaaccaaagacaccgagagcagtgtcttgctctcagacactgactcgggtttgggtacctaaataataaagcttggagaatgtgggcattgatcccactacctcttgcatgctaagcaagcgctctaccacttgagctaattccccatatcagggaagctttgtttatccttagtgggtggcctggaacacaggtgatttcagggccttcagcgggaaagcagggctctactaagagcagatcttctcattgatggcgcagggcaaggtgcagtggctactcattctctgcaaagaaggaggaaaaaagggaagaaggagaaagtcacaaagggaaaactcacgctgccaaaatgtgaagtttagggtattccaggacagaaaaagacacgtcccagcaaagaagacctatctagacctgcccagctaaagtgtcactgatttttaaaaaataattaaataattaaaaatgattaaatgattgtgtgtgtattgcatgtgtgtgtgtgtgtgtttataaaagtgggatggcattatcacttgttccttgtagctgagactctctgggggttgtgagatggtccagatttctggaaggcacaaaagggattctgaattaatatctgatgaatgaatccactcatttatttgtatttgttatgtgaatgaatgttacaggaatcacctggtgtggagaaaacagatggcaagactatgtgctagggtaaagcaagagctcacgtgtttttgtttttggttttttaatttagaaaaaaaatctgcttttcatatctggttttcctatttaaagctatgtgatttaaggaaaatggtttaactcctctgagctttagtgtcatctacaaaatttggataatgatactgagggaagctgaaaagccatatcaaccaacttatacaaaaaataataaacattcacttccatttctaatgcatggtgctgaaaaagtccttgtatgtggaatattgttcacctttaaggaacctgctctcaagagctgatgcgggactttttttagggcagttctgttgtctctggctgttttgttcatttaattggcacctacaagtctctttgaacattaaaataaaataaagattgtggaggaatagaatacaaacacatagtaaggtgagatttgcataacagagtatagtaaacgatttgtgcctgattctttttgcattctctttgaatcatttttagcctttattctaagtccccaattattgtcatccttttcccaacaagattgtttctctccgccacggacattctggtcagggtctctgcttaaccatcttgacctcctgaacactctgtttgtcctgataacctgatttatgctcaaatgatgctcttccataggacggcttcctgctttgcccaaagagcattcaatttttcaagctgtttagggctccttcctcacccagggtctatttgaaaccttagagggaaggctattctttccaggaagagaaccctgctgggttgtaacctcaatctgtaaatccactggggtaactggggttagctcagttactccagagcttgctctctgagaactggatggtgctgctacttcccataaaggctgaataaaaagaggcatctgcaggcaggagaaagcgctatggtcattgctggaagattccttctgaccattagctatctctctgacctggtgtgagaagggtgacaaaaatcggagacttgaaaacaggccaaaaaaaaaaaaatggattcaaaagaattttaaaagaatcatgcacaagttcttaattagattcttttatccaaatccattttgtctggaaaataataccttactacgtatctgtattctattcctccataatctattttattttattttaatgttcacaagaagctggatgctagctaccaaatgagcaaatcagccacgataacagaactgcactaaaatctctcatcagatattgatacagtcaagaccctcatgagtgcctatgatacaaattcagtgtgagaggccagctttccgcaaggagaaggcaaccaaagcggtagctaatactgagcagttcctattgcccagatccatttctaggtgctgagatccagccagagaatcccacagtcctcatttttcatatgaagaaacatgtgagtgattcaccaccccaatcctcatgtatcatcagttttcaaacaaagccaagtagcctcctgtgcaaaaagctctcctaacccccagttgccttgataggtaaaagtattcttatgacagtgctagaaaaacacgggcacaagtgttccggcaaggtgactagaaggcaaggctaaagttgtcaaggtgacaaagtccctgatggtcctcttgaaagctgaacgtgccacctcatatgtatatgtgtatgtgtggatgcatatgtgtatgttgtgtgtacacacctacacatatatctacaaatgcatgtgtgtatgcatgcatgtgtgtacacgtgcatgcgcacatgtatctgtatacatgtattatgtacacagtatgcatgtgtacatgtatgtgtgtctgtgcatgtgtagatgtatacatgcatgtacacatgcatctacatatgcatgtgtatgcctaaatgtgtgtacaagtgcgtgcatatgtgcactatacatatgtgtacattacgtgtgtgtatgtttctacacgtgtatctgca

SEQ ID NO: 11459 - RNA, 9823 nt, Homo sapiens
  source 1..9823: mol_type = other RNA
ctgaatagctgggactacaggtgcctgccaccacgcttggttaatttttgtatttttagtagagacggggtttcaccatgttggccaggctggtctcaacctcctgacgtcacgtgatcagcctaccttggccttccaaagtgctgggattacaggcatgagccacccctcctggcctgggtttaactattttattttatgacagggtctcactttgttgtccaggtaccggtgcgttctctgttcactgcaacctccacctcctgagttcaagcgatcctcccacctcagcctcctgagtagctggaactacagatgcataccaccacacccggctaatttttgtatttgttgtagagacaggttttcactgtgttgcctaggctggtctcaaactcctggtgtcaagggatccactgatctcggcctcccaaagtgctgggattacagaaatgagccaccacgtctggccctgggcttacctttcaagtcaactttgattcattgtcttccttgaaacaccacattcagtgattagtcaaataatgaacattattcttgcacaactcttttgaatctatcaattactttctactcatttagtacatattcactggggagatgctctgtgccagacactgtagtaagatcaggtaattcagaggaagtatagacaccccagacctcaaacgaagacaagataaatatggacaagggaagatccacctccacattcaccattttcagtctttctgtcatttccagctaaataacgtcttcaaaaatgtttcaaaataactaagtcactatttcaaactctttcaataatagcacccttctatacactggactactcttaattttctcattataacatgatcttgcttttcttttaatttttgtctttgctttctacctgaatttttattttgcattatgaaattgataggtccattactggatggcatggttcaattctccagtatgtctgttgatttgtgttccactaaatcttccaattactcagagaggagtgttaatgactgcaactataactggatttttctatttttacttggcgtatccaattttgtttatgagttttgaagctctgtgtcctcatatacatttgggacaatattctcctgaaaaattgacaatcataattatttaggaggcctcattattcctgaaaagtttctctgctttcaaatctactttgtctgattttatatatatacaccacagctgtctttgattaatgcttgcatgaggtatcttttcccactcttttctttcaatctgctctataacttttattcttatttataagtgtattgcaggtggctttctttagtcagcatatttatttttaacacattctgatgatctctagtttttacttaatgcatttagataatttacatataatgttattatagataagtttttagatagatctactatttaataatttattaaccttttttccctttgttttaattcttctatgttcctctgtctatcttgttttggtttatttcaatctggttgttaagtggtctagggattaccatatacatatataacttttcacagtatactaagaatcaatattttaccattcaagttgaatatagaaacttcatcaagagttagtcccattacatttacccttttatcttatgtatgtagtacatctagatacaatgacaactgcatcagataaagttacaatttttgctttcaaccatcaaacataccttaaggaactcaagagaagaataatagtctgttatgtctacccagacattttctatttctgcttttgttccttcattgatgatgttctaagtttccttctggtatcacttttcttatctcaaacctttgctaattcttttccagcagttttgctaggactgagaatgtatttatttaccttccaatgagaatgcatttatttgcctttatgtctggaagatacttttgctccacataccattctgggttgataatgtatttttcctttggtatttactgaatgttatgacatttttttctggctcctgggttcccgatgagaaatctacaatcattcatttggtattttatctttcatttccctttggctgctttcaaaattgttttgtgttttcttaattttccgcagtttgattatgatatgtcttgcaatgggtttcttttggtttatcctgcttgacatttactgaactttaaaaatctggtttatatcttttgagaaatttgatacattttcagccattaattcttcacagttttatcccacaaagacctctttgtcctcttacaataatgtgaatgtttccagattacaataatgtgaatgttagatttgttattttttatttgtccctgagcctctgttcagggacaataaaatcctcctttctttctataggtcagattctgtaggtattcttgttccgttttcaagttcattgactttttccttagtcttctgcatactgctattgagatcatccaattaagctttttatttcccctaatagttttggttaatactttttttaattcttaagtttaaattggtgtttacatattccaaatatttggtgagactttccaactttccattcacttcatgaatgctatcccgtaattctaggagcattgttataataactgctttaatgtatgtgtcagatgattttgacatatgtgtcctctcaatattgttatgcaaggattctctttgccatgtgaattaagatctccctggtttttcataatgctgaatattttggggcttgtaacctggacttctttggattatgtgatgagacactgtgtcttgttgaaatcttaaggataatattgctctttttgtttttgcaggcacacaattgccttgtatttaagctccaagtaccaaccagacttccatgtgttgttgtttcacagataactctatttgaaagccttgacactgcggatgagagatctctggagtgtgtgcaaccagtggtcagtgaggactggaaagtggaccattgtttagttcagtcctcaggctctttttaggtaagttgtttgggattagacccacttattcacagctggcaggtgcgtccacaagctcatgaacaactttatgggtttgctttctacagtatctgtccaggcacattctagttacttgacacatcctggtttcagtcctctcaccagaaagccagggctgtatttacccaggtggctctgccctgcacttttcacagttgcctcacattcaagctacaggcagaaacagggagaaaagagcaattgtttatgtcccttggtttcacagctcctcaaagaagcagaaaattaattacacggtagatctacactatactgaatgccaggagggagccgtcaccagccctgtattgttgctgctcctacatcttgaaccaaagcagcatcctgttctctgacttgggtttggagacctgagtgtttggagacccagggtctaaataataaagtttggagaatgtgggcatcgatcccactacctcttgcatgctaagcaagcgctctaccacttgagctaattcccccacatcaggggagctttattgatccttagtgggtggcctggaacacaggggatttcagggccttcagcgggaaagcagggctctactaagagcagatcttctcactgatggcccagggcaaggtgcagtggctactcattctctgcaaagaaggaagaggaaagggaacaaggagaaagtcaaaaagggaaaactcacactgccaaaatgtcaagtttagggtattccgggacagaaaaaggcacattccaggaaaggaggccctgcctagacctgcccatctaaagtgtcactgatttttaaaaaatgattaaataattaaaaatgattaaatgattttgtgtgtgtgtgttgtgtgtgtgtgtttataaaagtgagatagtattatcacttgttccttgtagctgagactctctggggattttgagatggtacagatttctggaaggcaaaaagctcctgttgttttcataactaggccctttcaggaatgaagccagcgtgctgaccactaccttaggaaacccctggggagtgcttctttcacttgcatctgagatataggttgcctccttgctaaggtgtgtcatgtacaagttacatgtccaactatatctcagaacaacaacaacaaaattacagagcagagccataaagaataagagacaagatcatatcagagtgtaagaatatgtaaaatattagagtgtaagaatcaaaattcagctatgcagagaaggagtggacatatggtggagaaaaccgggctgttcgtaggaattcctgtgtgaagaaataaacctgttcaatttaagtgctgtgtgtgtgtgtgtgtgtgtgtgtgtgtgtgaaatacacacggagggaagcagtgattgaaaagcctggccacttggagatatgttggtagagttttatgaaaactcccaagagtaattgaaaaaatcccaggcagaatgcttaaataattaaagcaacatgttagagaaaggtgtttagttttgaatgtcagagcttgaacatgagaaaatagaaattgaagagaaagagaaagaagtcataaagatattaaaggattgagatttacccgcatttatcgtgtcagctcccgaggtggacaacaggagtctttctgcagcgtcagtgcccatcacacttcctgctgcagaatacatcctccataaacaccatagcatggatgatgacagaggtgaatgaaaagaaagaaaaacattctggtgatgctgtgcaggaaggatctacagtatttgtcaagacattgggtggagagatttgagggagaggagacaaagacactgggaagtcttgagcctagtgtggtagacacaaaagagattctgaattaatagctgatgaatgaatccactcatttatttgtatttgttatgtgaatgaatgttacatgaatgacctggcatggagaaaacagatggtgagactatgtgctagggtaaagcaagagctcaagttttttttttttttttaatttagaaaaaaatctgcttttcatatctggttttcctatttaaaactatgtgatttgaggaaaatggtttaactcctctgagctttagtgtcatctacaaaatttggataatgatactgagggaagctgaaaagccgtatcaaccaacttatacaaaaaataataaacattcacttccatttctaatgcatggtgctgaaaaagtccttgtatgtggaatattgttcacctttaaggaacctgctctcaagagctgatgagggactttttttagtgcagttctgttgtcactggctgttgggctcatttagttggcaccaacaaatctctgtcttgctgctttttttcctcttgtggcccagtcatctagcttttcccttcttcagagatcttagtcactcttcttttccgtagtctccttaaggaactcaagggaagaataatagtctgttatgtctacccagacatgttctatttctgcttttgttccttcactgatgatgttctaagtttccttctggtatcatttttcttatctcaaatctttgctaattcttttccagcagtcttccgaatgttatgacattttttctggcccctatggttcctgatgcgaaatctacaatcattcatttggtagtttctctttcatttccctttggctgctttcaaaattgttttgtattttcttagttttcagcagtttgattatgatatgccttgctatgggtttctttgggtttatcctgattgacatttactgaactttaaaaatctggtttatatcttttgacaaatttgaaccattttcagctattaattgttcaaagttttatcccacaaagaccactttgtcctcttctttccagattacaataatgtgaatgttggatttgttattttttatttgtgcctgagcctctgttcagagacaataaaatcctcctttctctctatagttcagattatgtaggtattcgtgttctgttttcaagttcattgactttttccttagtcttctgcattcgattatggagatcctccaattaagctttttatttcccctaagagttttggttaatacatttttttaattcttaagtttaaattggtgtttatgtattcgaaatatttggtgagactttccaactttccattcacttcacgaatgttatccccgattctaggagcattgttataatatctgctttaatgtatgtgtcagatgattttgacatctgtgtcctctcaatattgttattcgaggattctctttgccatgtgaattaagatctccctgttttttcataatgctgaatattgtggggcttgtaacctggacttctttggattatgtgatgagacactgtgtcttgttgaaatcttaaggataatattgctatttttgtttttgcaggcacacaattgccttgtatttaagctccaagtaccaaccagactttcatgtgttgtcgtttcaaagataactctatttgaaagccttgacactgctgttcagagatctccaaagtgtgtgcaacccagtggtcagtgaggactggaaagtgggccattgcacagttcagctctcaggctctttttaggtaagttgttcgggattagagccacttattcacagctggcaggtgcgtccacaagctcatgaacaactttatggttttgctttctacagtatctgtccaggcacattctagttacttgacacatcttggtttcagtcctctcaccagaaagctggggctgtatttaaccaggtggctctgtcctccacttttcacaattgtctcacatttaggaccaagctgcaggcagaaacagggagaaaagagcagttttatatgtcctttggtttcacagctcctcgaagaaacagaaaattaattacacagtagatctacactatactgaatgccagcaggaagctgtcaccagtcctgtattgttgctgctcctatgtcttgaaccaaagacaccgagagcagtgtcttgctctcagacactgactcgggtttgggtacctaaataataaagcttggagaatgtgggcattgatcccactacctcttgcatgctaagcaagcgctctaccacttgagctaattccccatatcagggaagctttgtttatccttagtgggtggcctggaacacaggtgatttcagggccttcagcgggaaagcagggctctactaagagcagatcttctcattgatggcgcagggcaaggtgcagtggctactcattctctgcaaagaaggaggaaaaaagggaagaaggagaaagtcacaaagggaaaactcacgctgccaaaatgtgaagtttagggtattccaggacagaaaaagacacgtcccagcaaagaagacctatctagacctgcccagctaaagtgtcactgatttttaaaaaataattaaataattaaaaatgattaaatgattgtgtgtgtattgcatgtgtgtgtgtgtgtgtttataaaagtgggatggcattatcacttgttccttgtagctgagactctctgggggttgtgagatggtccagatttctggaaggcacaaaagggattctgaattaatatctgatgaatgaatccactcatttatttgtatttgttatgtgaatgaatgttacaggaatcacctggtgtggagaaaacagatggcaagactatgtgctagggtaaagcaagagctcacgtgtttttgtttttggttttttaatttagaaaaaaaatctgcttttcatatctggttttcctatttaaagctatgtgatttaaggaaaatggtttaactcctctgagctttagtgtcatctacaaaatttggataatgatactgagggaagctgaaaagccatatcaaccaacttatacaaaaaataataaacattcacttccatttctaatgcatggtgctgaaaaagtccttgtatgtggaatattgttcacctttaaggaacctgctctcaagagctgatgcgggactttttttagggcagttctgttgtctctggctgttttgttcatttaattggcacctacaagtctctttgaacattaaaataaaataaagattgtggaggaatagaatacaaacacatagtaaggtgagatttgcataacagagtatagtaaacgatttgtgcctgattctttttgcattctctttgaatcatttttagcctttattctaagtccccaattattgtcatccttttcccaacaagattgtttctctccgccacggacattctggtcagggtctctgcttaaccatcttgacctcctgaacactctgtttgtcctgataacctgatttatgctcaaatgatgctcttccataggacggcttcctgctttgcccaaagagcattcaatttttcaagctgtttagggctccttcctcacccagggtctatttgaaaccttagagggaaggctattctttccaggaagagaaccctgctgggttgtaacctcaatctgtaaatccactggggtaactggggttagctcagttactccagagcttgctctctgagaactggatggtgctgctacttcccataaaggctgaataaaaagaggcatctgcaggcaggagaaagcgctatggtcattgctggaagattccttctgaccattagctatctctctgacctggtgtgagaagggtgacaaaaatcggagacttgaaaacaggccaaaaaaaaaaaaatggattcaaaagaattttaaaagaatcatgcacaagttcttaattagattcttttatccaaatccattttgtctggaaaataataccttactacgtatctgtattctattcctccataatctattttattttattttaatgttcacaagaagctggatgctagctaccaaatgagcaaatcagccacgataacagaactgcactaaaatctctcatcagatattgatacagtcaagaccctcatgagtgcctatgatacaaattcagtgtgagaggccagctttccgcaaggagaaggcaaccaaagcggtagctaatactgagcagttcctattgcccagatccatttctaggtgctgagatccagccagagaatcccacagtcctcatttttcatatgaagaaacatgtgagtgattcaccaccccaatcctcatgtatcatcagttttcaaacaaagccaagtagcctcctgtgcaaaaagctctcctaacccccagttgccttgataggtaaaagtattcttatgacagtgctagaaaaacacgggcacaagtgttccggcaaggtgactagaaggcaaggctaaagttgtcaaggtgacaaagtccctgatggtcctcttgaaagctgaacgtgccacctcatatgtatatgtgtatgtgtggatgcatatgtgtatgttgtgtgtacacacctacacatatatctacaaatgcatgtgtgtatgcatgcatgtgtgtacacgtgcatgcgcacatgtatctgtatacatgtattatgtacacagtatgcatgtgtacatgtatgtgtgtctgtgcatgtgtagatgtatacatgcatgtacacatgcatctacatatgcatgtgtatgcctaaatgtgtgtacaagtgcgtgcatatgtgcactatacatatgtgtacattacgtgtgtgtatgtttctacacgtgtatctgcac

SEQ ID NO: 11460 - RNA, 9944 nt, Homo sapiens
  source 1..9944: mol_type = other RNA
ctgaatagctgggactacaggtgcctgccaccacgcttggttaatttttgtatttttagtagagacggggtttcaccatgttggccaggctggtctcaacctcctgacgtcacgtgatcagcctaccttggccttccaaagtgctgggattacaggcatgagccacccctcctggcctgggtttaactattttattttatgacagggtctcactttgttgtccaggtaccggtgcgttctctgttcactgcaacctccacctcctgagttcaagcgatcctcccacctcagcctcctgagtagctggaactacagatgcataccaccacacccggctaatttttgtatttgttgtagagacaggttttcactgtgttgcctaggctggtctcaaactcctggtgtcaagggatccactgatctcggcctcccaaagtgctgggattacagaaatgagccaccacgtctggccctgggcttacctttcaagtcaactttgattcattgtcttccttgaaacaccacattcagtgattagtcaaataatgaacattattcttgcacaactcttttgaatctatcaattactttctactcatttagtacatattcactggggagatgctctgtgccagacactgtagtaagatcaggtaattcagaggaagtatagacaccccagacctcaaacgaagacaagataaatatggacaagggaagatccacctccacattcaccattttcagtctttctgtcatttccagctaaataacgtcttcaaaaatgtttcaaaataactaagtcactatttcaaactctttcaataatagcacccttctatacactggactactcttaattttctcattataacatgatcttgcttttcttttaatttttgtctttgctttctacctgaatttttattttgcattatgaaattgataggtccattactggatggcatggttcaattctccagtatgtctgttgatttgtgttccactaaatcttccaattactcagagaggagtgttaatgactgcaactataactggatttttctatttttacttggcgtatccaattttgtttatgagttttgaagctctgtgtcctcatatacatttgggacaatattctcctgaaaaattgacaatcataattatttaggaggcctcattattcctgaaaagtttctctgctttcaaatctactttgtctgattttatatatatacaccacagctgtctttgattaatgcttgcatgaggtatcttttcccactcttttctttcaatctgctctataacttttattcttatttataagtgtattgcaggtggctttctttagtcagcatatttatttttaacacattctgatgatctctagtttttacttaatgcatttagataatttacatataatgttattatagataagtttttagatagatctactatttaataatttattaaccttttttccctttgttttaattcttctatgttcctctgtctatcttgttttggtttatttcaatctggttgttaagtggtctagggattaccatatacatatataacttttcacagtatactaagaatcaatattttaccattcaagttgaatatagaaacttcatcaagagttagtcccattacatttacccttttatcttatgtatgtagtacatctagatacaatgacaactgcatcagataaagttacaatttttgctttcaaccatcaaacataccttaaggaactcaagagaagaataatagtctgttatgtctacccagacattttctatttctgcttttgttccttcattgatgatgttctaagtttccttctggtatcacttttcttatctcaaacctttgctaattcttttccagcagttttgctaggactgagaatgtatttatttaccttccaatgagaatgcatttatttgcctttatgtctggaagatacttttgctccacataccattctgggttgataatgtatttttcctttggtatttactgaatgttatgacatttttttctggctcctgggttcccgatgagaaatctacaatcattcatttggtattttatctttcatttccctttggctgctttcaaaattgttttgtgttttcttaattttccgcagtttgattatgatatgtcttgcaatgggtttcttttggtttatcctgcttgacatttactgaactttaaaaatctggtttatatcttttgagaaatttgatacattttcagccattaattcttcacagttttatcccacaaagacctctttgtcctcttacaataatgtgaatgtttccagattacaataatgtgaatgttagatttgttattttttatttgtccctgagcctctgttcagggacaataaaatcctcctttctttctataggtcagattctgtaggtattcttgttccgttttcaagttcattgactttttccttagtcttctgcatactgctattgagatcatccaattaagctttttatttcccctaatagttttggttaatactttttttaattcttaagtttaaattggtgtttacatattccaaatatttggtgagactttccaactttccattcacttcatgaatgctatcccgtaattctaggagcattgttataataactgctttaatgtatgtgtcagatgattttgacatatgtgtcctctcaatattgttatgcaaggattctctttgccatgtgaattaagatctccctggtttttcataatgctgaatattttggggcttgtaacctggacttctttggattatgtgatgagacactgtgtcttgttgaaatcttaaggataatattgctctttttgtttttgcaggcacacaattgccttgtatttaagctccaagtaccaaccagacttccatgtgttgttgtttcacagataactctatttgaaagccttgacactgcggatgagagatctctggagtgtgtgcaaccagtggtcagtgaggactggaaagtggaccattgtttagttcagtcctcaggctctttttaggtaagttgtttgggattagacccacttattcacagctggcaggtgcgtccacaagctcatgaacaactttatgggtttgctttctacagtatctgtccaggcacattctagttacttgacacatcctggtttcagtcctctcaccagaaagccagggctgtatttacccaggtggctctgccctgcacttttcacagttgcctcacattcaagctacaggcagaaacagggagaaaagagcaattgtttatgtcccttggtttcacagctcctcaaagaagcagaaaattaattacacggtagatctacactatactgaatgccaggagggagccgtcaccagccctgtattgttgctgctcctacatcttgaaccaaagcagcatcctgttctctgacttgggtttggagacctgagtgtttggagacccagggtctaaataataaagtttggagaatgtgggcatcgatcccactacctcttgcatgctaagcaagcgctctaccacttgagctaattcccccacatcaggggagctttattgatccttagtgggtggcctggaacacaggggatttcagggccttcagcgggaaagcagggctctactaagagcagatcttctcactgatggcccagggcaaggtgcagtggctactcattctctgcaaagaaggaagaggaaagggaacaaggagaaagtcaaaaagggaaaactcacactgccaaaatgtcaagtttagggtattccgggacagaaaaaggcacattccaggaaaggaggccctgcctagacctgcccatctaaagtgtcactgatttttaaaaaatgattaaataattaaaaatgattaaatgattttgtgtgtgtgtgttgtgtgtgtgtgtttataaaagtgagatagtattatcacttgttccttgtagctgagactctctggggattttgagatggtacagatttctggaaggcaaaaagctcctgttgttttcataactaggccctttcaggaatgaagccagcgtgctgaccactaccttaggaaacccctggggagtgcttctttcacttgcatctgagatataggttgcctccttgctaaggtgtgtcatgtacaagttacatgtccaactatatctcagaacaacaacaacaaaattacagagcagagccataaagaataagagacaagatcatatcagagtgtaagaatatgtaaaatattagagtgtaagaatcaaaattcagctatgcagagaaggagtggacatatggtggagaaaaccgggctgttcgtaggaattcctgtgtgaagaaataaacctgttcaatttaagtgctgtgtgtgtgtgtgtgtgtgtgtgtgtgtgtgaaatacacacggagggaagcagtgattgaaaagcctggccacttggagatatgttggtagagttttatgaaaactcccaagagtaattgaaaaaatcccaggcagaatgcttaaataattaaagcaacatgttagagaaaggtgtttagttttgaatgtcagagcttgaacatgagaaaatagaaattgaagagaaagagaaagaagtcataaagatattaaaggattgagatttacccgcatttatcgtgtcagctcccgaggtggacaacaggagtctttctgcagcgtcagtgcccatcacacttcctgctgcagaatacatcctccataaacaccatagcatggatgatgacagaggtgaatgaaaagaaagaaaaacattctggtgatgctgtgcaggaaggatctacagtatttgtcaagacattgggtggagagatttgagggagaggagacaaagacactgggaagtcttgagcctagtgtggtagacacaaaagagattctgaattaatagctgatgaatgaatccactcatttatttgtatttgttatgtgaatgaatgttacatgaatgacctggcatggagaaaacagatggtgagactatgtgctagggtaaagcaagagctcaagttttttttttttttttaatttagaaaaaaatctgcttttcatatctggttttcctatttaaaactatgtgatttgaggaaaatggtttaactcctctgagctttagtgtcatctacaaaatttggataatgatactgagggaagctgaaaagccgtatcaaccaacttatacaaaaaataataaacattcacttccatttctaatgcatggtgctgaaaaagtccttgtatgtggaatattgttcacctttaaggaacctgctctcaagagctgatgagggactttttttagtgcagttctgttgtcactggctgttgggctcatttagttggcaccaacaaatctctgtcttgctgctttttttcctcttgtggcccagtcatctagcttttcccttcttcagagatcttagtcactcttcttttccgtagtctccttaaggaactcaagggaagaataatagtctgttatgtctacccagacatgttctatttctgcttttgttccttcactgatgatgttctaagtttccttctggtatcatttttcttatctcaaatctttgctaattcttttccagcagtcttcctaagaatgagaatgtatttacttaccttccactgagaatgcatttatttgcctttatgtctggaagatacttttgctccacatagcattctgggtcgatatgtctttttcttttgttacttaccgaatgttatgacattttttctggcccctatggttcctgatgcgaaatctacaatcattcatttggtagtttctctttcatttccctttggctgctttcaaaattgttttgtattttcttagttttcagcagtttgattatgatatgccttgctatgggtttctttgggtttatcctgattgacatttactgaactttaaaaatctggtttatatcttttgacaaatttgaaccattttcagctattaattgttcaaagttttatcccacaaagaccactttgtcctcttctttccagattacaataatgtgaatgttggatttgttattttttatttgtgcctgagcctctgttcagagacaataaaatcctcctttctctctatagttcagattatgtaggtattcgtgttctgttttcaagttcattgactttttccttagtcttctgcattcgattatggagatcctccaattaagctttttatttcccctaagagttttggttaatacatttttttaattcttaagtttaaattggtgtttatgtattcgaaatatttggtgagactttccaactttccattcacttcacgaatgttatccccgattctaggagcattgttataatatctgctttaatgtatgtgtcagatgattttgacatctgtgtcctctcaatattgttattcgaggattctctttgccatgtgaattaagatctccctgttttttcataatgctgaatattgtggggcttgtaacctggacttctttggattatgtgatgagacactgtgtcttgttgaaatcttaaggataatattgctatttttgtttttgcaggcacacaattgccttgtatttaagctccaagtaccaaccagactttcatgtgttgtcgtttcaaagataactctatttgaaagccttgacactgctgttcagagatctccaaagtgtgtgcaacccagtggtcagtgaggactggaaagtgggccattgcacagttcagctctcaggctctttttaggtaagttgttcgggattagagccacttattcacagctggcaggtgcgtccacaagctcatgaacaactttatggttttgctttctacagtatctgtccaggcacattctagttacttgacacatcttggtttcagtcctctcaccagaaagctggggctgtatttaaccaggtggctctgtcctccacttttcacaattgtctcacatttaggaccaagctgcaggcagaaacagggagaaaagagcagttttatatgtcctttggtttcacagctcctcgaagaaacagaaaattaattacacagtagatctacactatactgaatgccagcaggaagctgtcaccagtcctgtattgttgctgctcctatgtcttgaaccaaagacaccgagagcagtgtcttgctctcagacactgactcgggtttgggtacctaaataataaagcttggagaatgtgggcattgatcccactacctcttgcatgctaagcaagcgctctaccacttgagctaattccccatatcagggaagctttgtttatccttagtgggtggcctggaacacaggtgatttcagggccttcagcgggaaagcagggctctactaagagcagatcttctcattgatggcgcagggcaaggtgcagtggctactcattctctgcaaagaaggaggaaaaaagggaagaaggagaaagtcacaaagggaaaactcacgctgccaaaatgtgaagtttagggtattccaggacagaaaaagacacgtcccagcaaagaagacctatctagacctgcccagctaaagtgtcactgatttttaaaaaataattaaataattaaaaatgattaaatgattgtgtgtgtattgcatgtgtgtgtgtgtgtgtttataaaagtgggatggcattatcacttgttccttgtagctgagactctctgggggttgtgagatggtccagatttctggaaggcacaaaagggattctgaattaatatctgatgaatgaatccactcatttatttgtatttgttatgtgaatgaatgttacaggaatcacctggtgtggagaaaacagatggcaagactatgtgctagggtaaagcaagagctcacgtgtttttgtttttggttttttaatttagaaaaaaaatctgcttttcatatctggttttcctatttaaagctatgtgatttaaggaaaatggtttaactcctctgagctttagtgtcatctacaaaatttggataatgatactgagggaagctgaaaagccatatcaaccaacttatacaaaaaataataaacattcacttccatttctaatgcatggtgctgaaaaagtccttgtatgtggaatattgttcacctttaaggaacctgctctcaagagctgatgcgggactttttttagggcagttctgttgtctctggctgttttgttcatttaattggcacctacaagtctctttgaacattaaaataaaataaagattgtggaggaatagaatacaaacacatagtaaggtgagatttgcataacagagtatagtaaacgatttgtgcctgattctttttgcattctctttgaatcatttttagcctttattctaagtccccaattattgtcatccttttcccaacaagattgtttctctccgccacggacattctggtcagggtctctgcttaaccatcttgacctcctgaacactctgtttgtcctgataacctgatttatgctcaaatgatgctcttccataggacggcttcctgctttgcccaaagagcattcaatttttcaagctgtttagggctccttcctcacccagggtctatttgaaaccttagagggaaggctattctttccaggaagagaaccctgctgggttgtaacctcaatctgtaaatccactggggtaactggggttagctcagttactccagagcttgctctctgagaactggatggtgctgctacttcccataaaggctgaataaaaagaggcatctgcaggcaggagaaagcgctatggtcattgctggaagattccttctgaccattagctatctctctgacctggtgtgagaagggtgacaaaaatcggagacttgaaaacaggccaaaaaaaaaaaaatggattcaaaagaattttaaaagaatcatgcacaagttcttaattagattcttttatccaaatccattttgtctggaaaataataccttactacgtatctgtattctattcctccataatctattttattttattttaatgttcacaagaagctggatgctagctaccaaatgagcaaatcagccacgataacagaactgcactaaaatctctcatcagatattgatacagtcaagaccctcatgagtgcctatgatacaaattcagtgtgagaggccagctttccgcaaggagaaggcaaccaaagcggtagctaatactgagcagttcctattgcccagatccatttctaggtgctgagatccagccagagaatcccacagtcctcatttttcatatgaagaaacatgtgagtgattcaccaccccaatcctcatgtatcatcagttttcaaacaaagccaagtagcctcctgtgcaaaaagctctcctaacccccagttgccttgataggtaaaagtattcttatgacagtgctagaaaaacacgggcacaagtgttccggcaaggtgactagaaggcaaggctaaagttgtcaaggtgacaaagtccctgatggtcctcttgaaagctgaacgtgccacctcatatgtatatgtgtatgtgtggatgcatatgtgtatgttgtgtgtacacacctacacatatatctacaaatgcatgtgtgtatgcatgcatgtgtgtacacgtgcatgcgcacatgtatctgtatacatgtattatgtacacagtatgcatgtgtacatgtatgtgtgtctgtgcatgtgtagatgtatacatgcatgtacacatgcatctacatatgcatgtgtatgcctaaatgtgtgtacaagtgcgtgcatatgtgcactatacatatgtgtacattacgtgtgtgtatgtttctacacgtgtatctg

SEQ ID NO: 11461 - RNA, 5582 nt, Homo sapiens
  source 1..5582: mol_type = other RNA
ctgaatagctgggactacaggtgcctgccaccacgcttggttaatttttgtatttttagtagagacggggtttcaccatgttggccaggctggtctcaacctcctgacgtcacgtgatcagcctaccttggccttccaaagtgctgggattacaggcatgagccacccctcctggcctgggtttaactattttattttatgacagggtctcactttgttgtccaggtaccggtgcgttctctgttcactgcaacctccacctcctgagttcaagcgatcctcccacctcagcctcctgagtagctggaactacagatgcataccaccacacccggctaatttttgtatttgttgtagagacaggttttcactgtgttgcctaggctggtctcaaactcctggtgtcaagggatccactgatctcggcctcccaaagtgctgggattacagaaatgagccaccacgtctggccctgggcttacctttcaagtcaactttgattcattgtcttccttgaaacaccacattcagtgattagtcaaataatgaacattattcttgcacaactcttttgaatctatcaattactttctactcatttagtacatattcactggggagatgctctgtgccagacactgtagtaagatcaggtaattcagaggaagtatagacaccccagacctcaaacgaagacaagataaatatggacaagggaagatccacctccacattcaccattttcagtctttctgtcatttccagctaaataacgtcttcaaaaatgtttcaaaataactaagtcactatttcaaactctttcaataatagcacccttctatacactggactactcttaattttctcattataacatgatcttgcttttcttttaatttttgtctttgctttctacctgaatttttattttgcattatgaaattgataggtccattactggatggcatggttcaattctccagtatgtctgttgatttgtgttccactaaatcttccaattactcagagaggagtgttaatgactgcaactataactggatttttctatttttacttggcgtatccaattttgtttatgagttttgaagctctgtgtcctcatatacatttgggacaatattctcctgaaaaattgacaatcataattatttaggaggcctcattattcctgaaaagtttctctgctttcaaatctactttgtctgattttatatatatacaccacagctgtctttgattaatgcttgcatgaggtatcttttcccactcttttctttcaatctgctctataacttttattcttatttataagtgtattgcaggtggctttctttagtcagcatatttatttttaacacattctgatgatctctagtttttacttaatgcatttagataatttacatataatgttattatagataagtttttagatagatctactatttaataatttattaaccttttttccctttgttttaattcttctatgttcctctgtctatcttgttttggtttatttcaatctggttgttaagtggtctagggattaccatatacatatataacttttcacagtatactaagaatcaatattttaccattcaagttgaatatagaaacttcatcaagagttagtcccattacatttacccttttatcttatgtatgtagtacatctagatacaatgacaactgcatcagataaagttacaatttttgctttcaaccatcaaacataccttaaggaactcaagagaagaataatagtctgttatgtctacccagacattttctatttctgcttttgttccttcattgatgatgttctaagtttccttctggtatcacttttcttatctcaaacctttgctaattcttttccagcagttttgctaggactgagaatgtatttatttaccttccaatgagaatgcatttatttgcctttatgtctggaagatacttttgctccacataccattctgggttgataatgtatttttcctttggtatttactgaatgttatgacatttttttctggctcctgggttcccgatgagaaatctacaatcattcatttggtattttatctttcatttccctttggctgctttcaaaattgttttgtgttttcttaattttccgcagtttgattatgatatgtcttgcaatgggtttcttttggtttatcctgcttgacatttactgaactttaaaaatctggtttatatcttttgagaaatttgatacattttcagccattaattcttcacagttttatcccacaaagacctctttgtcctcttacaataatgtgaatgtttccagattacaataatgtgaatgttagatttgttattttttatttgtccctgagcctctgttcagggacaataaaatcctcctttctttctataggtcagattctgtaggtattcttgttccgttttcaagttcattgactttttccttagtcttctgcatactgctattgagatcatccaattaagctttttatttcccctaatagttttggttaatactttttttaattcttaagtttaaattggtgtttacatattccaaatatttggtgagactttccaactttccattcacttcatgaatgctatcccgtaattctaggagcattgttataataactgctttaatgtatgtgtcagatgattttgacatatgtgtcctctcaatattgttatgcaaggattctctttgccatgtgaattaagatctccctggtttttcataatgctgaatattttggggcttgtaacctggacttctttggattatgtgatgagacactgtgtcttgttgaaatcttaaggataatattgctctttttgtttttgcaggcacacaattgccttgtatttaagctccaagtaccaaccagacttccatgtgttgttgtttcacagataactctatttgaaagccttgacactgcggatgagagatctctggagtgtgtgcaaccagtggtcagtgaggactggaaagtggaccattgtttagttcagtcctcaggctctttttaggtaagttgtttgggattagacccacttattcacagctggcaggtgcgtccacaagctcatgaacaactttatgggtttgctttctacagtatctgtccaggcacattctagttacttgacacatcctggtttcagtcctctcaccagaaagccagggctgtatttacccaggtggctctgccctgcacttttcacagttgcctcacattcaagctacaggcagaaacagggagaaaagagcaattgtttatgtcccttggtttcacagctcctcaaagaagcagaaaattaattacacggtagatctacactatactgaatgccaggagggagccgtcaccagccctgtattgttgctgctcctacatcttgaaccaaagcagcatcctgttctctgacttgggtttggagacctgagtgtttggagacccagggtctaaataataaagtttggagaatgtgggcatcgatcccactacctcttgcatgctaagcaagcgctctaccacttgagctaattcccccacatcaggggagctttattgatccttagtgggtggcctggaacacaggggatttcagggccttcagcgggaaagcagggctctactaagagcagatcttctcactgatggcccagggcaaggtgcagtggctactcattctctgcaaagaaggaagaggaaagggaacaaggagaaagtcaaaaagggaaaactcacactgccaaaatgtcaagtttagggtattccgggacagaaaaaggcacattccaggaaaggaggccctgcctagacctgcccatctaaagtgtcactgatttttaaaaaatgattaaataattaaaaatgattaaatgattttgtgtgtgtgtgttgtgtgtgtgtgtttataaaagtgagatagtattatcacttgttccttgtagctgagactctctggggattttgagatggtacagatttctggaaggcaaaaagctcctgttgttttcataactaggccctttcaggaatgaagccagcgtgctgaccactaccttaggaaacccctggggagtgcttctttcacttgcatctgagatataggttgcctccttgctaaggtgtgtcatgtacaagttacatgtccaactatatctcagaacaacaacaacaaaattacagagcagagccataaagaataagagacaagatcatatcagagtgtaagaatatgtaaaatattagagtgtaagaatcaaaattcagctatgcagagaaggagtggacatatggtggagaaaaccgggctgttcgtaggaattcctgtgtgaagaaataaacctgttcaatttaagtgctgtgtgtgtgtgtgtgtgtgtgtgtgtgtgtgaaatacacacggagggaagcagtgattgaaaagcctggccacttggagatatgttggtagagttttatgaaaactcccaagagtaattgaaaaaatcccaggcagaatgcttaaataattaaagcaacatgttagagaaaggtgtttagttttgaatgtcagagcttgaacatgagaaaatagaaattgaagagaaagagaaagaagtcataaagatattaaaggattgagatttacccgcatttatcgtgtcagctcccgaggtggacaacaggagtctttctgcagcgtcagtgcccatcacacttcctgctgcagaatacatcctccataaacaccatagcatggatgatgacagaggtgaatgaaaagaaagaaaaacattctggtgatgctgtgcaggaaggatctacagtatttgtcaagacattgggtggagagatttgagggagaggagacaaagacactgggaagtcttgagcctagtgtggtagacacaaaagagattctgaattaatagctgatgaatgaatccactcatttatttgtatttgttatgtgaatgaatgttacatgaatgacctggcatggagaaaacagatggtgagactatgtgctagggtaaagcaagagctcaagttttttttttttttttaatttagaaaaaaatctgcttttcatatctggttttcctatttaaaactatgtgatttgaggaaaatggtttaactcctctgagctttagtgtcatctacaaaatttggataatgatactgagggaagctgaaaagccgtatcaaccaacttatacaaaaaataataaacattcacttccatttctaatgcatggtgctgaaaaagtccttgtatgtggaatattgttcacctttaaggaacctgctctcaagagctgatgagggactttttttagtgcagttctgttgtcactggctgttgggctcatttagttggcaccaacaaatctctgtcttgctgctttttttcctcttgtggcccagtcatctagcttttcccttcttcagagatcttagtcactcttcttttccgtagtctctttgttgtccaggcaccggtgcaatctctgttcactgcaacctccg

SEQ ID NO: 11462 - RNA, 9441 nt, Homo sapiens
  source 1..9441: mol_type = other RNA
ctgaatagctgggactacaggtgcctgccaccacgcttggttaatttttgtatttttagtagagacggggtttcaccatgttggccaggctggtctcaacctcctgacgtcacgtgatcagcctaccttggccttccaaagtgctgggattacaggcatgagccacccctcctggcctgggtttaactattttattttatgacagggtctcactttgttgtccaggtaccggtgcgttctctgttcactgcaacctccacctcctgagttcaagcgatcctcccacctcagcctcctgagtagctggaactacagatgcataccaccacacccggctaatttttgtatttgttgtagagacaggttttcactgtgttgcctaggctggtctcaaactcctggtgtcaagggatccactgatctcggcctcccaaagtgctgggattacagaaatgagccaccacgtctggccctgggcttacctttcaagtcaactttgattcattgtcttccttgaaacaccacattcagtgattagtcaaataatgaacattattcttgcacaactcttttgaatctatcaattactttctactcatttagtacatattcactggggagatgctctgtgccagacactgtagtaagatcaggtaattcagaggaagtatagacaccccagacctcaaacgaagacaagataaatatggacaagggaagatccacctccacattcaccattttcagtctttctgtcatttccagctaaataacgtcttcaaaaatgtttcaaaataactaagtcactatttcaaactctttcaataatagcacccttctatacactggactactcttaattttctcattataacatgatcttgcttttcttttaatttttgtctttgctttctacctgaatttttattttgcattatgaaattgataggtccattactggatggcatggttcaattctccagtatgtctgttgatttgtgttccactaaatcttccaattactcagagaggagtgttaatgactgcaactataactggatttttctatttttacttggcgtatccaattttgtttatgagttttgaagctctgtgtcctcatatacatttgggacaatattctcctgaaaaattgacaatcataattatttaggaggcctcattattcctgaaaagtttctctgctttcaaatctactttgtctgattttatatatatacaccacagctgtctttgattaatgcttgcatgaggtatcttttcccactcttttctttcaatctgctctataacttttattcttatttataagtgtattgcaggtggctttctttagtcagcatatttatttttaacacattctgatgatctctagtttttacttaatgcatttagataatttacatataatgttattatagataagtttttagatagatctactatttaataatttattaaccttttttccctttgttttaattcttctatgttcctctgtctatcttgttttggtttatttcaatctggttgttaagtggtctagggattaccatatacatatataacttttcacagtatactaagaatcaatattttaccattcaagttgaatatagaaacttcatcaagagttagtcccattacatttacccttttatcttatgtatgtagtacatctagatacaatgacaactgcatcagataaagttacaatttttgctttcaaccatcaaacataccttaaggaactcaagagaagaataatagtctgttatgtctacccagacattttctatttctgcttttgttccttcattgatgatgttctaagtttccttctggtatcacttttcttatctcaaacctttgctaattcttttccagcagttttgctaggactgagaatgtatttatttaccttccaatgagaatgcatttatttgcctttatgtctggaagatacttttgctccacataccattctgggttgataatgtatttttcctttggtatttactgaatgttatgacatttttttctggctcctgggttcccgatgagaaatctacaatcattcatttggtattttatctttcatttccctttggctgctttcaaaattgttttgtgttttcttaattttccgcagtttgattatgatatgtcttgcaatgggtttcttttggtttatcctgcttgacatttactgaactttaaaaatctggtttatatcttttgagaaatttgatacattttcagccattaattcttcacagttttatcccacaaagacctctttgtcctcttacaataatgtgaatgtttccagattacaataatgtgaatgttagatttgttattttttatttgtccctgagcctctgttcagggacaataaaatcctcctttctttctataggtcagattctgtaggtattcttgttccgttttcaagttcattgactttttccttagtcttctgcatactgctattgagatcatccaattaagctttttatttcccctaatagttttggttaatactttttttaattcttaagtttaaattggtgtttacatattccaaatatttggtgagactttccaactttccattcacttcatgaatgctatcccgtaattctaggagcattgttataataactgctttaatgtatgtgtcagatgattttgacatatgtgtcctctcaatattgttatgcaaggattctctttgccatgtgaattaagatctccctggtttttcataatgctgaatattttggggcttgtaacctggacttctttggattatgtgatgagacactgtgtcttgttgaaatcttaaggataatattgctctttttgtttttgcaggcacacaattgccttgtatttaagctccaagtaccaaccagacttccatgtgttgttgtttcacagataactctatttgaaagccttgacactgcggatgagagatctctggagtgtgtgcaaccagtggtcagtgaggactggaaagtggaccattgtttagttcagtcctcaggctctttttaggtaagttgtttgggattagacccacttattcacagctggcaggtgcgtccacaagctcatgaacaactttatgggtttgctttctacagtatctgtccaggcacattctagttacttgacacatcctggtttcagtcctctcaccagaaagccagggctgtatttacccaggtggctctgccctgcacttttcacagttgcctcacattcaagctacaggcagaaacagggagaaaagagcaattgtttatgtcccttggtttcacagctcctcaaagaagcagaaaattaattacacggtagatctacactatactgaatgccaggagggagccgtcaccagccctgtattgttgctgctcctacatcttgaaccaaagcagcatcctgttctctgacttgggtttggagacctgagtgtttggagacccagggtctaaataataaagtttggagaatgtgggcatcgatcccactacctcttgcatgctaagcaagcgctctaccacttgagctaattcccccacatcaggggagctttattgatccttagtgggtggcctggaacacaggggatttcagggccttcagcgggaaagcagggctctactaagagcagatcttctcactgatggcccagggcaaggtgcagtggctactcattctctgcaaagaaggaagaggaaagggaacaaggagaaagtcaaaaagggaaaactcacactgccaaaatgtcaagtttagggtattccgggacagaaaaaggcacattccaggaaaggaggccctgcctagacctgcccatctaaagtgtcactgatttttaaaaaatgattaaataattaaaaatgattaaatgattttgtgtgtgtgtgttgtgtgtgtgtgtttataaaagtgagatagtattatcacttgttccttgtagctgagactctctggggattttgagatggtacagatttctggaaggcaaaaagctcctgttgttttcataactaggccctttcaggaatgaagccagcgtgctgaccactaccttaggaaacccctggggagtgcttctttcacttgcatctgagatataggttgcctccttgctaaggtgtgtcatgtacaagttacatgtccaactatatctcagaacaacaacaacaaaattacagagcagagccataaagaataagagacaagatcatatcagagtgtaagaatatgtaaaatattagagtgtaagaatcaaaattcagctatgcagagaaggagtggacatatggtggagaaaaccgggctgttcgtaggaattcctgtgtgaagaaataaacctgttcaatttaagtgctgtgtgtgtgtgtgtgtgtgtgtgtgtgtgtgaaatacacacggagggaagcagtgattgaaaagcctggccacttggagatatgttggtagagttttatgaaaactcccaagagtaattgaaaaaatcccaggcagaatgcttaaataattaaagcaacatgttagagaaaggtgtttagttttgaatgtcagagcttgaacatgagaaaatagaaattgaagagaaagagaaagaagtcataaagatattaaaggattgagatttacccgcatttatcgtgtcagctcccgaggtggacaacaggagtctttctgcagcgtcagtgcccatcacacttcctgctgcagaatacatcctccataaacaccatagcatggatgatgacagaggtgaatgaaaagaaagaaaaacattctggtgatgctgtgcaggaaggatctacagtatttgtcaagacattgggtggagagatttgagggagaggagacaaagacactgggaagtcttgagcctgtcttgctgctttttttcctcttgtggcccagtcatctagcttttcccttcttcagagatcttagtcactcttcttttccgtagtctccttaaggaactcaagggaagaataatagtctgttatgtctacccagacatgttctatttctgcttttgttccttcactgatgatgttctaagtttccttctggtatcatttttcttatctcaaatctttgctaattcttttccagcagtcttcctaagaatgagaatgtatttacttaccttccactgagaatgcatttatttgcctttatgtctggaagatacttttgctccacatagcattctgggtcgatatgtctttttcttttgttacttaccgaatgttatgacattttttctggcccctatggttcctgatgcgaaatctacaatcattcatttggtagtttctctttcatttccctttggctgctttcaaaattgttttgtattttcttagttttcagcagtttgattatgatatgccttgctatgggtttctttgggtttatcctgattgacatttactgaactttaaaaatctggtttatatcttttgacaaatttgaaccattttcagctattaattgttcaaagttttatcccacaaagaccactttgtcctcttctttccagattacaataatgtgaatgttggatttgttattttttatttgtgcctgagcctctgttcagagacaataaaatcctcctttctctctatagttcagattatgtaggtattcgtgttctgttttcaagttcattgactttttccttagtcttctgcattcgattatggagatcctccaattaagctttttatttcccctaagagttttggttaatacatttttttaattcttaagtttaaattggtgtttatgtattcgaaatatttggtgagactttccaactttccattcacttcacgaatgttatccccgattctaggagcattgttataatatctgctttaatgtatgtgtcagatgattttgacatctgtgtcctctcaatattgttattcgaggattctctttgccatgtgaattaagatctccctgttttttcataatgctgaatattgtggggcttgtaacctggacttctttggattatgtgatgagacactgtgtcttgttgaaatcttaaggataatattgctatttttgtttttgcaggcacacaattgccttgtatttaagctccaagtaccaaccagactttcatgtgttgtcgtttcaaagataactctatttgaaagccttgacactgctgttcagagatctccaaagtgtgtgcaacccagtggtcagtgaggactggaaagtgggccattgcacagttcagctctcaggctctttttaggtaagttgttcgggattagagccacttattcacagctggcaggtgcgtccacaagctcatgaacaactttatggttttgctttctacagtatctgtccaggcacattctagttacttgacacatcttggtttcagtcctctcaccagaaagctggggctgtatttaaccaggtggctctgtcctccacttttcacaattgtctcacatttaggaccaagctgcaggcagaaacagggagaaaagagcagttttatatgtcctttggtttcacagctcctcgaagaaacagaaaattaattacacagtagatctacactatactgaatgccagcaggaagctgtcaccagtcctgtattgttgctgctcctatgtcttgaaccaaagacaccgagagcagtgtcttgctctcagacactgactcgggtttgggtacctaaataataaagcttggagaatgtgggcattgatcccactacctcttgcatgctaagcaagcgctctaccacttgagctaattccccatatcagggaagctttgtttatccttagtgggtggcctggaacacaggtgatttcagggccttcagcgggaaagcagggctctactaagagcagatcttctcattgatggcgcagggcaaggtgcagtggctactcattctctgcaaagaaggaggaaaaaagggaagaaggagaaagtcacaaagggaaaactcacgctgccaaaatgtgaagtttagggtattccaggacagaaaaagacacgtcccagcaaagaagacctatctagacctgcccagctaaagtgtcactgatttttaaaaaataattaaataattaaaaatgattaaatgattgtgtgtgtattgcatgtgtgtgtgtgtgtgtttataaaagtgggatggcattatcacttgttccttgtagctgagactctctgggggttgtgagatggtccagatttctggaaggcacaaaagggattctgaattaatatctgatgaatgaatccactcatttatttgtatttgttatgtgaatgaatgttacaggaatcacctggtgtggagaaaacagatggcaagactatgtgctagggtaaagcaagagctcacgtgtttttgtttttggttttttaatttagaaaaaaaatctgcttttcatatctggttttcctatttaaagctatgtgatttaaggaaaatggtttaactcctctgagctttagtgtcatctacaaaatttggataatgatactgagggaagctgaaaagccatatcaaccaacttatacaaaaaataataaacattcacttccatttctaatgcatggtgctgaaaaagtccttgtatgtggaatattgttcacctttaaggaacctgctctcaagagctgatgcgggactttttttagggcagttctgttgtctctggctgttttgttcatttaattggcacctacaagtctctttgaacattaaaataaaataaagattgtggaggaatagaatacaaacacatagtaaggtgagatttgcataacagagtatagtaaacgatttgtgcctgattctttttgcattctctttgaatcatttttagcctttattctaagtccccaattattgtcatccttttcccaacaagattgtttctctccgccacggacattctggtcagggtctctgcttaaccatcttgacctcctgaacactctgtttgtcctgataacctgatttatgctcaaatgatgctcttccataggacggcttcctgctttgcccaaagagcattcaatttttcaagctgtttagggctccttcctcacccagggtctatttgaaaccttagagggaaggctattctttccaggaagagaaccctgctgggttgtaacctcaatctgtaaatccactggggtaactggggttagctcagttactccagagcttgctctctgagaactggatggtgctgctacttcccataaaggctgaataaaaagaggcatctgcaggcaggagaaagcgctatggtcattgctggaagattccttctgaccattagctatctctctgacctggtgtgagaagggtgacaaaaatcggagacttgaaaacaggccaaaaaaaaaaaaatggattcaaaagaattttaaaagaatcatgcacaagttcttaattagattcttttatccaaatccattttgtctggaaaataataccttactacgtatctgtattctattcctccataatctattttattttattttaatgttcacaagaagctggatgctagctaccaaatgagcaaatcagccacgataacagaactgcactaaaatctctcatcagatattgatacagtcaagaccctcatgagtgcctatgatacaaattcagtgtgagaggccagctttccgcaaggagaaggcaaccaaagcggtagctaatactgagcagttcctattgcccagatccatttctaggtgctgagatccagccagagaatcccacagtcctcatttttcatatgaagaaacatgtgagtgattcaccaccccaatcctcatgtatcatcagttttcaaacaaagccaagtagcctcctgtgcaaaaagctctcctaacccccagttgccttgataggtaaaagtattcttatgacagtgctagaaaaacacgggcacaagtgttccggcaaggtgactagaaggcaaggctaaagttgtcaaggtgacaaagtccctgatggtcctcttgaaagctgaacgtgccacctcatatgtatatgtgtatgtgtggatgcatatgtgtatgttgtgtgtacacacctacacatatatctacaaatgcatgtgtgtatgcatgcatgtgtgtacacgtgcatgcgcacatgtatctgtatacatgtattatgtacacagtatgcatgtgtacatgtatgtgtgtctgtgcatgtgtagatgtatacatgcatgtacacatgcatctacatatgcatgtgtatgcctaaatgtgtgtacaagtgcgtgcatatgtgcactatacatatgtgtacattacgtgtgtgtatgtttctacacgtgtatctg

SEQ ID NO: 11463 - RNA, 9285 nt, Homo sapiens
  source 1..9285: mol_type = other RNA
ctgaatagctgggactacaggtgcctgccaccacgcttggttaatttttgtatttttagtagagacggggtttcaccatgttggccaggctggtctcaacctcctgacgtcacgtgatcagcctaccttggccttccaaagtgctgggattacaggcatgagccacccctcctggcctgggtttaactattttattttatgacagggtctcactttgttgtccaggtaccggtgcgttctctgttcactgcaacctccacctcctgagttcaagcgatcctcccacctcagcctcctgagtagctggaactacagatgcataccaccacacccggctaatttttgtatttgttgtagagacaggttttcactgtgttgcctaggctggtctcaaactcctggtgtcaagggatccactgatctcggcctcccaaagtgctgggattacagaaatgagccaccacgtctggccctgggcttacctttcaagtcaactttgattcattgtcttccttgaaacaccacattcagtgattagtcaaataatgaacattattcttgcacaactcttttgaatctatcaattactttctactcatttagtacatattcactggggagatgctctgtgccagacactgtagtaagatcaggtaattcagaggaagtatagacaccccagacctcaaacgaagacaagataaatatggacaagggaagatccacctccacattcaccattttcagtctttctgtcatttccagctaaataacgtcttcaaaaatgtttcaaaataactaagtcactatttcaaactctttcaataatagcacccttctatacactggactactcttaattttctcattataacatgatcttgcttttcttttaatttttgtctttgctttctacctgaatttttattttgcattatgaaattgataggtccattactggatggcatggttcaattctccagtatgtctgttgatttgtgttccactaaatcttccaattactcagagaggagtgttaatgactgcaactataactggatttttctatttttacttggcgtatccaattttgtttatgagttttgaagctctgtgtcctcatatacatttgggacaatattctcctgaaaaattgacaatcataattatttaggaggcctcattattcctgaaaagtttctctgctttcaaatctactttgtctgattttatatatatacaccacagctgtctttgattaatgcttgcatgaggtatcttttcccactcttttctttcaatctgctctataacttttattcttatttataagtgtattgcaggtggctttctttagtcagcatatttatttttaacacattctgatgatctctagtttttacttaatgcatttagataatttacatataatgttattatagataagtttttagatagatctactatttaataatttattaaccttttttccctttgttttaattcttctatgttcctctgtctatcttgttttggtttatttcaatctggttgttaagtggtctagggattaccatatacatatataacttttcacagtatactaagaatcaatattttaccattcaagttgaatatagaaacttcatcaagagttagtcccattacatttacccttttatcttatgtatgtagtacatctagatacaatgacaactgcatcagataaagttacaatttttgctttcaaccatcaaacataccttaaggaactcaagagaagaataatagtctgttatgtctacccagacattttctatttctgcttttgttccttcattgatgatgttctaagtttccttctggtatcacttttcttatctcaaacctttgctaattcttttccagcagttttgctaggactgagaatgtatttatttaccttccaatgagaatgcatttatttgcctttatgtctggaagatacttttgctccacataccattctgggttgataatgtatttttcctttggtatttactgaatgttatgacatttttttctggctcctgggttcccgatgagaaatctacaatcattcatttggtattttatctttcatttccctttggctgctttcaaaattgttttgtgttttcttaattttccgcagtttgattatgatatgtcttgcaatgggtttcttttggtttatcctgcttgacatttactgaactttaaaaatctggtttatatcttttgagaaatttgatacattttcagccattaattcttcacagttttatcccacaaagacctctttgtcctcttacaataatgtgaatgtttccagattacaataatgtgaatgttagatttgttattttttatttgtccctgagcctctgttcagggacaataaaatcctcctttctttctataggtcagattctgtaggtattcttgttccgttttcaagttcattgactttttccttagtcttctgcatactgctattgagatcatccaattaagctttttatttcccctaatagttttggttaatactttttttaattcttaagtttaaattggtgtttacatattccaaatatttggtgagactttccaactttccattcacttcatgaatgctatcccgtaattctaggagcattgttataataactgctttaatgtatgtgtcagatgattttgacatatgtgtcctctcaatattgttatgcaaggattctctttgccatgtgaattaagatctccctggtttttcataatgctgaatattttggggcttgtaacctggacttctttggattatgtgatgagacactgtgtcttgttgaaatcttaaggataatattgctctttttgtttttgcaggcacacaattgccttgtatttaagctccaagtaccaaccagacttccatgtgttgttgtttcacagataactctatttgaaagccttgacactgcggatgagagatctctggagtgtgtgcaaccagtggtcagtgaggactggaaagtggaccattgtttagttcagtcctcaggctctttttaggtaagttgtttgggattagacccacttattcacagctggcaggtgcgtccacaagctcatgaacaactttatgggtttgctttctacagtatctgtccaggcacattctagttacttgacacatcctggtttcagtcctctcaccagaaagccagggctgtatttacccaggtggctctgccctgcacttttcacagttgcctcacattcaagctacaggcagaaacagggagaaaagagcaattgtttatgtcccttggtttcacagctcctcaaagaagcagaaaattaattacacggtagatctacactatactgaatgccaggagggagccgtcaccagccctgtattgttgctgctcctacatcttgaaccaaagcagcatcctgttctctgacttgggtttggagacctgagtgtttggagacccagggtctaaataataaagtttggagaatgtgggcatcgatcccactacctcttgcatgctaagcaagcgctctaccacttgagctaattcccccacatcaggggagctttattgatccttagtgggtggcctggaacacaggggatttcagggccttcagcgggaaagcagggctctactaagagcagatcttctcactgatggcccagggcaaggtgcagtggctactcattctctgcaaagaaggaagaggaaagggaacaaggagaaagtcaaaaagggaaaactcacactgccaaaatgtcaagtttagggtattccgggacagaaaaaggcacattccaggaaaggaggccctgcctagacctgcccatctaaagtgtcactgatttttaaaaaatgattaaataattaaaaatgattaaatgattttgtgtgtgtgtgttgtgtgtgtgtgtttataaaagtgagatagtattatcacttgttccttgtagctgagactctctggggattttgagatggtacagatttctggaaggcaaaaagctcctgttgttttcataactaggccctttcaggaatgaagccagcgtgctgaccactaccttaggaaacccctggggagtgcttctttcacttgcatctgagatataggttgcctccttgctaaggtgtgtcatgtacaagttacatgtccaactatatctcagaacaacaacaacaaaattacagagcagagccataaagaataagagacaagatcatatcagagtgtaagaatatgtaaaatattagagtgtaagaatcaaaattcagctatgcagagaaggagtggacatatggtggagaaaaccgggctgttcgtaggaattcctgtgtgaagaaataaacctgttcaatttaagtgctgtgtgtgtgtgtgtgtgtgtgtgtgtgtgtgaaatacacacggagggaagcagtgattgaaaagcctggccacttggagatatgttggtagagttttatgaaaactcccaagagtaattgaaaaaatcccaggcagaatgcttaaataattaaagcaacatgttagagaaaggtgtttagttttgaatgtcagagcttgaacatgagaaaatagaaattgaagagaaagagaaagaagtcataaagatattaaaggattgagatttacccgcatttatcgtgtcagctcccgaggtggacaacaggagtctttctgcagcgtcagtgcccatcacacttcctgctgcagaatacatcctgtcttgctgctttttttcctcttgtggcccagtcatctagcttttcccttcttcagagatcttagtcactcttcttttccgtagtctccttaaggaactcaagggaagaataatagtctgttatgtctacccagacatgttctatttctgcttttgttccttcactgatgatgttctaagtttccttctggtatcatttttcttatctcaaatctttgctaattcttttccagcagtcttcctaagaatgagaatgtatttacttaccttccactgagaatgcatttatttgcctttatgtctggaagatacttttgctccacatagcattctgggtcgatatgtctttttcttttgttacttaccgaatgttatgacattttttctggcccctatggttcctgatgcgaaatctacaatcattcatttggtagtttctctttcatttccctttggctgctttcaaaattgttttgtattttcttagttttcagcagtttgattatgatatgccttgctatgggtttctttgggtttatcctgattgacatttactgaactttaaaaatctggtttatatcttttgacaaatttgaaccattttcagctattaattgttcaaagttttatcccacaaagaccactttgtcctcttctttccagattacaataatgtgaatgttggatttgttattttttatttgtgcctgagcctctgttcagagacaataaaatcctcctttctctctatagttcagattatgtaggtattcgtgttctgttttcaagttcattgactttttccttagtcttctgcattcgattatggagatcctccaattaagctttttatttcccctaagagttttggttaatacatttttttaattcttaagtttaaattggtgtttatgtattcgaaatatttggtgagactttccaactttccattcacttcacgaatgttatccccgattctaggagcattgttataatatctgctttaatgtatgtgtcagatgattttgacatctgtgtcctctcaatattgttattcgaggattctctttgccatgtgaattaagatctccctgttttttcataatgctgaatattgtggggcttgtaacctggacttctttggattatgtgatgagacactgtgtcttgttgaaatcttaaggataatattgctatttttgtttttgcaggcacacaattgccttgtatttaagctccaagtaccaaccagactttcatgtgttgtcgtttcaaagataactctatttgaaagccttgacactgctgttcagagatctccaaagtgtgtgcaacccagtggtcagtgaggactggaaagtgggccattgcacagttcagctctcaggctctttttaggtaagttgttcgggattagagccacttattcacagctggcaggtgcgtccacaagctcatgaacaactttatggttttgctttctacagtatctgtccaggcacattctagttacttgacacatcttggtttcagtcctctcaccagaaagctggggctgtatttaaccaggtggctctgtcctccacttttcacaattgtctcacatttaggaccaagctgcaggcagaaacagggagaaaagagcagttttatatgtcctttggtttcacagctcctcgaagaaacagaaaattaattacacagtagatctacactatactgaatgccagcaggaagctgtcaccagtcctgtattgttgctgctcctatgtcttgaaccaaagacaccgagagcagtgtcttgctctcagacactgactcgggtttgggtacctaaataataaagcttggagaatgtgggcattgatcccactacctcttgcatgctaagcaagcgctctaccacttgagctaattccccatatcagggaagctttgtttatccttagtgggtggcctggaacacaggtgatttcagggccttcagcgggaaagcagggctctactaagagcagatcttctcattgatggcgcagggcaaggtgcagtggctactcattctctgcaaagaaggaggaaaaaagggaagaaggagaaagtcacaaagggaaaactcacgctgccaaaatgtgaagtttagggtattccaggacagaaaaagacacgtcccagcaaagaagacctatctagacctgcccagctaaagtgtcactgatttttaaaaaataattaaataattaaaaatgattaaatgattgtgtgtgtattgcatgtgtgtgtgtgtgtgtttataaaagtgggatggcattatcacttgttccttgtagctgagactctctgggggttgtgagatggtccagatttctggaaggcacaaaagggattctgaattaatatctgatgaatgaatccactcatttatttgtatttgttatgtgaatgaatgttacaggaatcacctggtgtggagaaaacagatggcaagactatgtgctagggtaaagcaagagctcacgtgtttttgtttttggttttttaatttagaaaaaaaatctgcttttcatatctggttttcctatttaaagctatgtgatttaaggaaaatggtttaactcctctgagctttagtgtcatctacaaaatttggataatgatactgagggaagctgaaaagccatatcaaccaacttatacaaaaaataataaacattcacttccatttctaatgcatggtgctgaaaaagtccttgtatgtggaatattgttcacctttaaggaacctgctctcaagagctgatgcgggactttttttagggcagttctgttgtctctggctgttttgttcatttaattggcacctacaagtctctttgaacattaaaataaaataaagattgtggaggaatagaatacaaacacatagtaaggtgagatttgcataacagagtatagtaaacgatttgtgcctgattctttttgcattctctttgaatcatttttagcctttattctaagtccccaattattgtcatccttttcccaacaagattgtttctctccgccacggacattctggtcagggtctctgcttaaccatcttgacctcctgaacactctgtttgtcctgataacctgatttatgctcaaatgatgctcttccataggacggcttcctgctttgcccaaagagcattcaatttttcaagctgtttagggctccttcctcacccagggtctatttgaaaccttagagggaaggctattctttccaggaagagaaccctgctgggttgtaacctcaatctgtaaatccactggggtaactggggttagctcagttactccagagcttgctctctgagaactggatggtgctgctacttcccataaaggctgaataaaaagaggcatctgcaggcaggagaaagcgctatggtcattgctggaagattccttctgaccattagctatctctctgacctggtgtgagaagggtgacaaaaatcggagacttgaaaacaggccaaaaaaaaaaaaatggattcaaaagaattttaaaagaatcatgcacaagttcttaattagattcttttatccaaatccattttgtctggaaaataataccttactacgtatctgtattctattcctccataatctattttattttattttaatgttcacaagaagctggatgctagctaccaaatgagcaaatcagccacgataacagaactgcactaaaatctctcatcagatattgatacagtcaagaccctcatgagtgcctatgatacaaattcagtgtgagaggccagctttccgcaaggagaaggcaaccaaagcggtagctaatactgagcagttcctattgcccagatccatttctaggtgctgagatccagccagagaatcccacagtcctcatttttcatatgaagaaacatgtgagtgattcaccaccccaatcctcatgtatcatcagttttcaaacaaagccaagtagcctcctgtgcaaaaagctctcctaacccccagttgccttgataggtaaaagtattcttatgacagtgctagaaaaacacgggcacaagtgttccggcaaggtgactagaaggcaaggctaaagttgtcaaggtgacaaagtccctgatggtcctcttgaaagctgaacgtgccacctcatatgtatatgtgtatgtgtggatgcatatgtgtatgttgtgtgtacacacctacacatatatctacaaatgcatgtgtgtatgcatgcatgtgtgtacacgtgcatgcgcacatgtatctgtatacatgtattatgtacacagtatgcatgtgtacatgtatgtgtgtctgtgcatgtgtagatgtatacatgcatgtacacatgcatctacatatgcatgtgtatgcctaaatgtgtgtacaagtgcgtgcatatgtgcactatacatatgtgtacattacgtgtgtgtatgtttctacacgtgtatctg

SEQ ID NO: 11464 - RNA, 8251 nt, Homo sapiens
  source 1..8251: mol_type = other RNA
ctgaatagctgggactacaggtgcctgccaccacgcttggttaatttttgtatttttagtagagacggggtttcaccatgttggccaggctggtctcaacctcctgacgtcacgtgatcagcctaccttggccttccaaagtgctgggattacaggcatgagccacccctcctggcctgggtttaactattttattttatgacagggtctcactttgttgtccaggtaccggtgcgttctctgttcactgcaacctccacctcctgagttcaagcgatcctcccacctcagcctcctgagtagctggaactacagatgcataccaccacacccggctaatttttgtatttgttgtagagacaggttttcactgtgttgcctaggctggtctcaaactcctggtgtcaagggatccactgatctcggcctcccaaagtgctgggattacagaaatgagccaccacgtctggccctgggcttacctttcaagtcaactttgattcattgtcttccttgaaacaccacattcagtgattagtcaaataatgaacattattcttgcacaactcttttgaatctatcaattactttctactcatttagtacatattcactggggagatgctctgtgccagacactgtagtaagatcaggtaattcagaggaagtatagacaccccagacctcaaacgaagacaagataaatatggacaagggaagatccacctccacattcaccattttcagtctttctgtcatttccagctaaataacgtcttcaaaaatgtttcaaaataactaagtcactatttcaaactctttcaataatagcacccttctatacactggactactcttaattttctcattataacatgatcttgcttttcttttaatttttgtctttgctttctacctgaatttttattttgcattatgaaattgataggtccattactggatggcatggttcaattctccagtatgtctgttgatttgtgttccactaaatcttccaattactcagagaggagtgttaatgactgcaactataactggatttttctatttttacttggcgtatccaattttgtttatgagttttgaagctctgtgtcctcatatacatttgggacaatattctcctgaaaaattgacaatcataattatttaggaggcctcattattcctgaaaagtttctctgctttcaaatctactttgtctgattttatatatatacaccacagctgtctttgattaatgcttgcatgaggtatcttttcccactcttttctttcaatctgctctataacttttattcttatttataagtgtattgcaggtggctttctttagtcagcatatttatttttaacacattctgatgatctctagtttttacttaatgcatttagataatttacatataatgttattatagataagtttttagatagatctactatttaataatttattaaccttttttccctttgttttaattcttctatgttcctctgtctatcttgttttggtttatttcaatctggttgttaagtggtctagggattaccatatacatatataacttttcacagtatactaagaatcaatattttaccattcaagttgaatatagaaacttcatcaagagttagtcccattacatttacccttttatcttatgtatgtagtacatctagatacaatgacaactgcatcagataaagttacaatttttgctttcaaccatcaaacataccttaaggaactcaagagaagaataatagtctgttatgtctacccagacattttctatttctgcttttgttccttcattgatgatgttctaagtttccttctggtatcacttttcttatctcaaacctttgctaattcttttccagcagttttgctaggactgagaatgtatttatttaccttccaatgagaatgcatttatttgcctttatgtctggaagatacttttgctccacataccattctgggttgataatgtatttttcctttggtatttactgaatgttatgacatttttttctggctcctgggttcccgatgagaaatctacaatcattcatttggtattttatctttcatttccctttggctgctttcaaaattgttttgtgttttcttaattttccgcagtttgattatgatatgtcttgcaatgggtttcttttggtttatcctgcttgacatttactgaactttaaaaatctggtttatatcttttgagaaatttgatacattttcagccattaattcttcacagttttatcccacaaagacctctttgtcctcttacaataatgtgaatgtttccagattacaataatgtgaatgttagatttgttattttttatttgtccctgagcctctgttcagggacaataaaatcctcctttctttctataggtcagattctgtaggtattcttgttccgttttcaagttcattgactttttccttagtcttctgcatactgctattgagatcatccaattaagctttttatttcccctaatagttttggttaatactttttttaattcttaagtttaaattggtgtttacatattccaaatatttggtgagactttccaactttccattcacttcatgaatgctatcccgtaattctaggagcattgttataataactgctttaatgtatgtgtcagatgattttgacatatgtgtcctctcaatattgttatgcaaggattctctttgccatgtgaattaagatctccctggtttttcataatgctgaatattttggggcttgtaacctggacttctttggattatgtgatgagacactgtgtcttgttgaaatcttaaggataatattgctctttttgtttttgcaggcacacaattgccttgtatttaagctccaagtaccaaccagacttccatgtgttgttgtttcacagataactctatttgaaagccttgacactgcggatgagagatctctggagtgtgtgcaaccagtggtcagtgaggactggaaagtggaccattgtttagttcagtcctcaggctctttttaggtaagttgtttgggattagacccacttattcacagctggcaggtgcgtccacaagctcatgaacaactttatgggtttgctttctacagtatctgtccaggcacattctagttacttgacacatcctggtttcagtcctctcaccagaaagccagggctgtatttacccaggtggctctgccctgcacttttcacagttgcctcacattcaagctacaggcagaaacagggagaaaagagcaattgtttatgtcccttggtttcacagctcctcaaagaagcagaaaattaattacacggtagatctacactatactgaatgccaggagggagccgtcaccagccctgtattgttgctgctcctacatcttgaaccaaagcagcatcctgttctctgacttgggtttggagacctgagtgtttggagacccagggtctaaataataaagtttggagaatgtgggcatcgatcccactacctcttgcatgctaagcaagcgctctaccacttgagctaattcccccacatcaggggagctttattgatccttagtgggtggcctggaacacaggggatttcagggccttcagcgggaaagcagggctctactaagagcagatcttctcactgatggcccagggcaaggtgcagtggctactcattctctgtcttgctgctttttttcctcttgtggcccagtcatctagcttttcccttcttcagagatcttagtcactcttcttttccgtagtctccttaaggaactcaagggaagaataatagtctgttatgtctacccagacatgttctatttctgcttttgttccttcactgatgatgttctaagtttccttctggtatcatttttcttatctcaaatctttgctaattcttttccagcagtcttcctaagaatgagaatgtatttacttaccttccactgagaatgcatttatttgcctttatgtctggaagatacttttgctccacatagcattctgggtcgatatgtctttttcttttgttacttaccgaatgttatgacattttttctggcccctatggttcctgatgcgaaatctacaatcattcatttggtagtttctctttcatttccctttggctgctttcaaaattgttttgtattttcttagttttcagcagtttgattatgatatgccttgctatgggtttctttgggtttatcctgattgacatttactgaactttaaaaatctggtttatatcttttgacaaatttgaaccattttcagctattaattgttcaaagttttatcccacaaagaccactttgtcctcttctttccagattacaataatgtgaatgttggatttgttattttttatttgtgcctgagcctctgttcagagacaataaaatcctcctttctctctatagttcagattatgtaggtattcgtgttctgttttcaagttcattgactttttccttagtcttctgcattcgattatggagatcctccaattaagctttttatttcccctaagagttttggttaatacatttttttaattcttaagtttaaattggtgtttatgtattcgaaatatttggtgagactttccaactttccattcacttcacgaatgttatccccgattctaggagcattgttataatatctgctttaatgtatgtgtcagatgattttgacatctgtgtcctctcaatattgttattcgaggattctctttgccatgtgaattaagatctccctgttttttcataatgctgaatattgtggggcttgtaacctggacttctttggattatgtgatgagacactgtgtcttgttgaaatcttaaggataatattgctatttttgtttttgcaggcacacaattgccttgtatttaagctccaagtaccaaccagactttcatgtgttgtcgtttcaaagataactctatttgaaagccttgacactgctgttcagagatctccaaagtgtgtgcaacccagtggtcagtgaggactggaaagtgggccattgcacagttcagctctcaggctctttttaggtaagttgttcgggattagagccacttattcacagctggcaggtgcgtccacaagctcatgaacaactttatggttttgctttctacagtatctgtccaggcacattctagttacttgacacatcttggtttcagtcctctcaccagaaagctggggctgtatttaaccaggtggctctgtcctccacttttcacaattgtctcacatttaggaccaagctgcaggcagaaacagggagaaaagagcagttttatatgtcctttggtttcacagctcctcgaagaaacagaaaattaattacacagtagatctacactatactgaatgccagcaggaagctgtcaccagtcctgtattgttgctgctcctatgtcttgaaccaaagacaccgagagcagtgtcttgctctcagacactgactcgggtttgggtacctaaataataaagcttggagaatgtgggcattgatcccactacctcttgcatgctaagcaagcgctctaccacttgagctaattccccatatcagggaagctttgtttatccttagtgggtggcctggaacacaggtgatttcagggccttcagcgggaaagcagggctctactaagagcagatcttctcattgatggcgcagggcaaggtgcagtggctactcattctctgcaaagaaggaggaaaaaagggaagaaggagaaagtcacaaagggaaaactcacgctgccaaaatgtgaagtttagggtattccaggacagaaaaagacacgtcccagcaaagaagacctatctagacctgcccagctaaagtgtcactgatttttaaaaaataattaaataattaaaaatgattaaatgattgtgtgtgtattgcatgtgtgtgtgtgtgtgtttataaaagtgggatggcattatcacttgttccttgtagctgagactctctgggggttgtgagatggtccagatttctggaaggcacaaaagggattctgaattaatatctgatgaatgaatccactcatttatttgtatttgttatgtgaatgaatgttacaggaatcacctggtgtggagaaaacagatggcaagactatgtgctagggtaaagcaagagctcacgtgtttttgtttttggttttttaatttagaaaaaaaatctgcttttcatatctggttttcctatttaaagctatgtgatttaaggaaaatggtttaactcctctgagctttagtgtcatctacaaaatttggataatgatactgagggaagctgaaaagccatatcaaccaacttatacaaaaaataataaacattcacttccatttctaatgcatggtgctgaaaaagtccttgtatgtggaatattgttcacctttaaggaacctgctctcaagagctgatgcgggactttttttagggcagttctgttgtctctggctgttttgttcatttaattggcacctacaagtctctttgaacattaaaataaaataaagattgtggaggaatagaatacaaacacatagtaaggtgagatttgcataacagagtatagtaaacgatttgtgcctgattctttttgcattctctttgaatcatttttagcctttattctaagtccccaattattgtcatccttttcccaacaagattgtttctctccgccacggacattctggtcagggtctctgcttaaccatcttgacctcctgaacactctgtttgtcctgataacctgatttatgctcaaatgatgctcttccataggacggcttcctgctttgcccaaagagcattcaatttttcaagctgtttagggctccttcctcacccagggtctatttgaaaccttagagggaaggctattctttccaggaagagaaccctgctgggttgtaacctcaatctgtaaatccactggggtaactggggttagctcagttactccagagcttgctctctgagaactggatggtgctgctacttcccataaaggctgaataaaaagaggcatctgcaggcaggagaaagcgctatggtcattgctggaagattccttctgaccattagctatctctctgacctggtgtgagaagggtgacaaaaatcggagacttgaaaacaggccaaaaaaaaaaaaatggattcaaaagaattttaaaagaatcatgcacaagttcttaattagattcttttatccaaatccattttgtctggaaaataataccttactacgtatctgtattctattcctccataatctattttattttattttaatgttcacaagaagctggatgctagctaccaaatgagcaaatcagccacgataacagaactgcactaaaatctctcatcagatattgatacagtcaagaccctcatgagtgcctatgatacaaattcagtgtgagaggccagctttccgcaaggagaaggcaaccaaagcggtagctaatactgagcagttcctattgcccagatccatttctaggtgctgagatccagccagagaatcccacagtcctcatttttcatatgaagaaacatgtgagtgattcaccaccccaatcctcatgtatcatcagttttcaaacaaagccaagtagcctcctgtgcaaaaagctctcctaacccccagttgccttgataggtaaaagtattcttatgacagtgctagaaaaacacgggcacaagtgttccggcaaggtgactagaaggcaaggctaaagttgtcaaggtgacaaagtccctgatggtcctcttgaaagctgaacgtgccacctcatatgtatatgtgtatgtgtggatgcatatgtgtatgttgtgtgtacacacctacacatatatctacaaatgcatgtgtgtatgcatgcatgtgtgtacacgtgcatgcgcacatgtatctgtatacatgtattatgtacacagtatgcatgtgtacatgtatgtgtgtctgtgcatgtgtagatgtatacatgcatgtacacatgcatctacatatgcatgtgtatgcctaaatgtgtgtacaagtgcgtgcatatgtgcactatacatatgtgtacattacgtgtgtgtatgtttctacacgtgtatctg

SEQ ID NO: 11465 - RNA, 7798 nt, Homo sapiens
  source 1..7798: mol_type = other RNA
ctgaatagctgggactacaggtgcctgccaccacgcttggttaatttttgtatttttagtagagacggggtttcaccatgttggccaggctggtctcaacctcctgacgtcacgtgatcagcctaccttggccttccaaagtgctgggattacaggcatgagccacccctcctggcctgggtttaactattttattttatgacagggtctcactttgttgtccaggtaccggtgcgttctctgttcactgcaacctccacctcctgagttcaagcgatcctcccacctcagcctcctgagtagctggaactacagatgcataccaccacacccggctaatttttgtatttgttgtagagacaggttttcactgtgttgcctaggctggtctcaaactcctggtgtcaagggatccactgatctcggcctcccaaagtgctgggattacagaaatgagccaccacgtctggccctgggcttacctttcaagtcaactttgattcattgtcttccttgaaacaccacattcagtgattagtcaaataatgaacattattcttgcacaactcttttgaatctatcaattactttctactcatttagtacatattcactggggagatgctctgtgccagacactgtagtaagatcaggtaattcagaggaagtatagacaccccagacctcaaacgaagacaagataaatatggacaagggaagatccacctccacattcaccattttcagtctttctgtcatttccagctaaataacgtcttcaaaaatgtttcaaaataactaagtcactatttcaaactctttcaataatagcacccttctatacactggactactcttaattttctcattataacatgatcttgcttttcttttaatttttgtctttgctttctacctgaatttttattttgcattatgaaattgataggtccattactggatggcatggttcaattctccagtatgtctgttgatttgtgttccactaaatcttccaattactcagagaggagtgttaatgactgcaactataactggatttttctatttttacttggcgtatccaattttgtttatgagttttgaagctctgtgtcctcatatacatttgggacaatattctcctgaaaaattgacaatcataattatttaggaggcctcattattcctgaaaagtttctctgctttcaaatctactttgtctgattttatatatatacaccacagctgtctttgattaatgcttgcatgaggtatcttttcccactcttttctttcaatctgctctataacttttattcttatttataagtgtattgcaggtggctttctttagtcagcatatttatttttaacacattctgatgatctctagtttttacttaatgcatttagataatttacatataatgttattatagataagtttttagatagatctactatttaataatttattaaccttttttccctttgttttaattcttctatgttcctctgtctatcttgttttggtttatttcaatctggttgttaagtggtctagggattaccatatacatatataacttttcacagtatactaagaatcaatattttaccattcaagttgaatatagaaacttcatcaagagttagtcccattacatttacccttttatcttatgtatgtagtacatctagatacaatgacaactgcatcagataaagttacaatttttgctttcaaccatcaaacataccttaaggaactcaagagaagaataatagtctgttatgtctacccagacattttctatttctgcttttgttccttcattgatgatgttctaagtttccttctggtatcacttttcttatctcaaacctttgctaattcttttccagcagttttgctaggactgagaatgtatttatttaccttccaatgagaatgcatttatttgcctttatgtctggaagatacttttgctccacataccattctgggttgataatgtatttttcctttggtatttactgaatgttatgacatttttttctggctcctgggttcccgatgagaaatctacaatcattcatttggtattttatctttcatttccctttggctgctttcaaaattgttttgtgttttcttaattttccgcagtttgattatgatatgtcttgcaatgggtttcttttggtttatcctgcttgacatttactgaactttaaaaatctggtttatatcttttgagaaatttgatacattttcagccattaattcttcacagttttatcccacaaagacctctttgtcctcttacaataatgtgaatgtttccagattacaataatgtgaatgttagatttgttattttttatttgtccctgagcctctgttcagggacaataaaatcctcctttctttctataggtcagattctgtaggtattcttgttccgttttcaagttcattgactttttccttagtcttctgcatactgctattgagatcatccaattaagctttttatttcccctaatagttttggttaatactttttttaattcttaagtttaaattggtgtttacatattccaaatatttggtgagactttccaactttccattcacttcatgaatgctatcccgtaattctaggagcattgttataataactgctttaatgtatgtgtcagatgattttgacatatgtgtcctctcaatattgttatgcaaggattctctttgccatgtgaattaagatctccctggtttttcataatgctgaatattttggggcttgtaacctggacttctttggattatgtgatgagacactgtgtcttgttgaaatcttaaggataatattgctctttttgtttttgcaggcacacaattgccttgtatttaagctccaagtaccaaccagacttccatgtgttgttgtttcacagataactctatttgaaagccttgacactgcggatgagagatctctggagtgtgtgcaaccagtggtcagtgaggactggaaagtggaccattgtttagttcagtcctcaggctctttttaggtaagttgtttgggattagacccacttattcacagctggcaggtgcgtccacaagctcatgaacaactttatgggtttgctttctacagtatctgtccaggcacattctagttacttgacacatcctggtttcagtcctctcaccagaaagccagggctgtatttacccaggtggctctgccctgcacttttcacagttgcctcacattcaagctgtcttgctgctttttttcctcttgtggcccagtcatctagcttttcccttcttcagagatcttagtcactcttcttttccgtagtctccttaaggaactcaagggaagaataatagtctgttatgtctacccagacatgttctatttctgcttttgttccttcactgatgatgttctaagtttccttctggtatcatttttcttatctcaaatctttgctaattcttttccagcagtcttcctaagaatgagaatgtatttacttaccttccactgagaatgcatttatttgcctttatgtctggaagatacttttgctccacatagcattctgggtcgatatgtctttttcttttgttacttaccgaatgttatgacattttttctggcccctatggttcctgatgcgaaatctacaatcattcatttggtagtttctctttcatttccctttggctgctttcaaaattgttttgtattttcttagttttcagcagtttgattatgatatgccttgctatgggtttctttgggtttatcctgattgacatttactgaactttaaaaatctggtttatatcttttgacaaatttgaaccattttcagctattaattgttcaaagttttatcccacaaagaccactttgtcctcttctttccagattacaataatgtgaatgttggatttgttattttttatttgtgcctgagcctctgttcagagacaataaaatcctcctttctctctatagttcagattatgtaggtattcgtgttctgttttcaagttcattgactttttccttagtcttctgcattcgattatggagatcctccaattaagctttttatttcccctaagagttttggttaatacatttttttaattcttaagtttaaattggtgtttatgtattcgaaatatttggtgagactttccaactttccattcacttcacgaatgttatccccgattctaggagcattgttataatatctgctttaatgtatgtgtcagatgattttgacatctgtgtcctctcaatattgttattcgaggattctctttgccatgtgaattaagatctccctgttttttcataatgctgaatattgtggggcttgtaacctggacttctttggattatgtgatgagacactgtgtcttgttgaaatcttaaggataatattgctatttttgtttttgcaggcacacaattgccttgtatttaagctccaagtaccaaccagactttcatgtgttgtcgtttcaaagataactctatttgaaagccttgacactgctgttcagagatctccaaagtgtgtgcaacccagtggtcagtgaggactggaaagtgggccattgcacagttcagctctcaggctctttttaggtaagttgttcgggattagagccacttattcacagctggcaggtgcgtccacaagctcatgaacaactttatggttttgctttctacagtatctgtccaggcacattctagttacttgacacatcttggtttcagtcctctcaccagaaagctggggctgtatttaaccaggtggctctgtcctccacttttcacaattgtctcacatttaggaccaagctgcaggcagaaacagggagaaaagagcagttttatatgtcctttggtttcacagctcctcgaagaaacagaaaattaattacacagtagatctacactatactgaatgccagcaggaagctgtcaccagtcctgtattgttgctgctcctatgtcttgaaccaaagacaccgagagcagtgtcttgctctcagacactgactcgggtttgggtacctaaataataaagcttggagaatgtgggcattgatcccactacctcttgcatgctaagcaagcgctctaccacttgagctaattccccatatcagggaagctttgtttatccttagtgggtggcctggaacacaggtgatttcagggccttcagcgggaaagcagggctctactaagagcagatcttctcattgatggcgcagggcaaggtgcagtggctactcattctctgcaaagaaggaggaaaaaagggaagaaggagaaagtcacaaagggaaaactcacgctgccaaaatgtgaagtttagggtattccaggacagaaaaagacacgtcccagcaaagaagacctatctagacctgcccagctaaagtgtcactgatttttaaaaaataattaaataattaaaaatgattaaatgattgtgtgtgtattgcatgtgtgtgtgtgtgtgtttataaaagtgggatggcattatcacttgttccttgtagctgagactctctgggggttgtgagatggtccagatttctggaaggcacaaaagggattctgaattaatatctgatgaatgaatccactcatttatttgtatttgttatgtgaatgaatgttacaggaatcacctggtgtggagaaaacagatggcaagactatgtgctagggtaaagcaagagctcacgtgtttttgtttttggttttttaatttagaaaaaaaatctgcttttcatatctggttttcctatttaaagctatgtgatttaaggaaaatggtttaactcctctgagctttagtgtcatctacaaaatttggataatgatactgagggaagctgaaaagccatatcaaccaacttatacaaaaaataataaacattcacttccatttctaatgcatggtgctgaaaaagtccttgtatgtggaatattgttcacctttaaggaacctgctctcaagagctgatgcgggactttttttagggcagttctgttgtctctggctgttttgttcatttaattggcacctacaagtctctttgaacattaaaataaaataaagattgtggaggaatagaatacaaacacatagtaaggtgagatttgcataacagagtatagtaaacgatttgtgcctgattctttttgcattctctttgaatcatttttagcctttattctaagtccccaattattgtcatccttttcccaacaagattgtttctctccgccacggacattctggtcagggtctctgcttaaccatcttgacctcctgaacactctgtttgtcctgataacctgatttatgctcaaatgatgctcttccataggacggcttcctgctttgcccaaagagcattcaatttttcaagctgtttagggctccttcctcacccagggtctatttgaaaccttagagggaaggctattctttccaggaagagaaccctgctgggttgtaacctcaatctgtaaatccactggggtaactggggttagctcagttactccagagcttgctctctgagaactggatggtgctgctacttcccataaaggctgaataaaaagaggcatctgcaggcaggagaaagcgctatggtcattgctggaagattccttctgaccattagctatctctctgacctggtgtgagaagggtgacaaaaatcggagacttgaaaacaggccaaaaaaaaaaaaatggattcaaaagaattttaaaagaatcatgcacaagttcttaattagattcttttatccaaatccattttgtctggaaaataataccttactacgtatctgtattctattcctccataatctattttattttattttaatgttcacaagaagctggatgctagctaccaaatgagcaaatcagccacgataacagaactgcactaaaatctctcatcagatattgatacagtcaagaccctcatgagtgcctatgatacaaattcagtgtgagaggccagctttccgcaaggagaaggcaaccaaagcggtagctaatactgagcagttcctattgcccagatccatttctaggtgctgagatccagccagagaatcccacagtcctcatttttcatatgaagaaacatgtgagtgattcaccaccccaatcctcatgtatcatcagttttcaaacaaagccaagtagcctcctgtgcaaaaagctctcctaacccccagttgccttgataggtaaaagtattcttatgacagtgctagaaaaacacgggcacaagtgttccggcaaggtgactagaaggcaaggctaaagttgtcaaggtgacaaagtccctgatggtcctcttgaaagctgaacgtgccacctcatatgtatatgtgtatgtgtggatgcatatgtgtatgttgtgtgtacacacctacacatatatctacaaatgcatgtgtgtatgcatgcatgtgtgtacacgtgcatgcgcacatgtatctgtatacatgtattatgtacacagtatgcatgtgtacatgtatgtgtgtctgtgcatgtgtagatgtatacatgcatgtacacatgcatctacatatgcatgtgtatgcctaaatgtgtgtacaagtgcgtgcatatgtgcactatacatatgtgtacattacgtgtgtgtatgtttctacacgtgtatctg

SEQ ID NO: 11466 - RNA, 7898 nt, Homo sapiens
  source 1..7898: mol_type = other RNA
ctgaatagctgggactacaggtgcctgccaccacgcttggttaatttttgtatttttagtagagacggggtttcaccatgttggccaggctggtctcaacctcctgacgtcacgtgatcagcctaccttggccttccaaagtgctgggattacaggcatgagccacccctcctggcctgggtttaactattttattttatgacagggtctcactttgttgtccaggtaccggtgcgttctctgttcactgcaacctccacctcctgagttcaagcgatcctcccacctcagcctcctgagtagctggaactacagatgcataccaccacacccggctaatttttgtatttgttgtagagacaggttttcactgtgttgcctaggctggtctcaaactcctggtgtcaagggatccactgatctcggcctcccaaagtgctgggattacagaaatgagccaccacgtctggccctgggcttacctttcaagtcaactttgattcattgtcttccttgaaacaccacattcagtgattagtcaaataatgaacattattcttgcacaactcttttgaatctatcaattactttctactcatttagtacatattcactggggagatgctctgtgccagacactgtagtaagatcaggtaattcagaggaagtatagacaccccagacctcaaacgaagacaagataaatatggacaagggaagatccacctccacattcaccattttcagtctttctgtcatttccagctaaataacgtcttcaaaaatgtttcaaaataactaagtcactatttcaaactctttcaataatagcacccttctatacactggactactcttaattttctcattataacatgatcttgcttttcttttaatttttgtctttgctttctacctgaatttttattttgcattatgaaattgataggtccattactggatggcatggttcaattctccagtatgtctgttgatttgtgttccactaaatcttccaattactcagagaggagtgttaatgactgcaactataactggatttttctatttttacttggcgtatccaattttgtttatgagttttgaagctctgtgtcctcatatacatttgggacaatattctcctgaaaaattgacaatcataattatttaggaggcctcattattcctgaaaagtttctctgctttcaaatctactttgtctgattttatatatatacaccacagctgtctttgattaatgcttgcatgaggtatcttttcccactcttttctttcaatctgctctataacttttattcttatttataagtgtattgcaggtggctttctttagtcagcatatttatttttaacacattctgatgatctctagtttttacttaatgcatttagataatttacatataatgttattatagataagtttttagatagatctactatttaataatttattaaccttttttccctttgttttaattcttctatgttcctctgtctatcttgttttggtttatttcaatctggttgttaagtggtctagggattaccatatacatatataacttttcacagtatactaagaatcaatattttaccattcaagttgaatatagaaacttcatcaagagttagtcccattacatttacccttttatcttatgtatgtagtacatctagatacaatgacaactgcatcagataaagttacaatttttgctttcaaccatcaaacataccttaaggaactcaagagaagaataatagtctgttatgtctacccagacattttctatttctgcttttgttccttcattgatgatgttctaagtttccttctggtatcacttttcttatctcaaacctttgctaattcttttccagcagttttgctaggactgagaatgtatttatttaccttccaatgagaatgcatttatttgcctttatgtctggaagatacttttgctccacataccattctgggttgataatgtatttttcctttggtatttactgaatgttatgacatttttttctggctcctgggttcccgatgagaaatctacaatcattcatttggtattttatctttcatttccctttggctgctttcaaaattgttttgtgttttcttaattttccgcagtttgattatgatatgtcttgcaatgggtttcttttggtttatcctgcttgacatttactgaactttaaaaatctggtttatatcttttgagaaatttgatacattttcagccattaattcttcacagttttatcccacaaagacctctttgtcctcttacaataatgtgaatgtttccagattacaataatgtgaatgttagatttgttattttttatttgtccctgagcctctgttcagggacaataaaatcctcctttctttctataggtcagattctgtaggtattcttgttccgttttcaagttcattgactttttccttagtcttctgcatactgctattgagatcatccaattaagctttttatttcccctaatagttttggttaatactttttttaattcttaagtttaaattggtgtttacatattccaaatatttggtgagactttccaactttccattcacttcatgaatgctatcccgtaattctaggagcattgttataataactgctttaatgtatgtgtcagatgattttgacatatgtgtcctctcaatattgttatgcaaggattctctttgccatgtgaattaagatctccctggtttttcataatgctgaatattttggggcttgtaacctggacttctttggattatgtgatgagacactgtgtcttgttgaaatcttaaggataatattgctctttttgtttttgcaggcacacaattgccttgtatttaagctccaagtaccaaccagacttccatgtgttgttgtttcacagataactctatttgaaagccttgacactgcggatgagagatctctggagtgtgtgcaaccagtggtcagtgaggactggaaagtggaccattgtttagttcagtcctcaggctctttttaggtaagttgtttgggattagacccacttattcacagctggcaggtgcgtccacaagctcatgaacaactttatgggtttgctttctacagtatctgtccaggcacattctagttacttgacacatcctggtttcagtcctctcaccagaaagccagggctgtatttacccaggtggctctgccctgcacttttcacagttgcctcacattcaagctttaaggaacctgctctcaagagctgatgagggactttttttagtgcagttctgttgtcactggctgttgggctcatttagttggcaccaacaaatctctgtcttgctgctttttttcctcttgtggcccagtcatctagcttttcccttcttcagagatcttagtcactcttcttttccgtagtctccttaaggaactcaagggaagaataatagtctgttatgtctacccagacatgttctatttctgcttttgttccttcactgatgatgttctaagtttccttctggtatcatttttcttatctcaaatctttgctaattcttttccagcagtcttcctaagaatgagaatgtatttacttaccttccactgagaatgcatttatttgcctttatgtctggaagatacttttgctccacatagcattctgggtcgatatgtctttttcttttgttacttaccgaatgttatgacattttttctggcccctatggttcctgatgcgaaatctacaatcattcatttggtagtttctctttcatttccctttggctgctttcaaaattgttttgtattttcttagttttcagcagtttgattatgatatgccttgctatgggtttctttgggtttatcctgattgacatttactgaactttaaaaatctggtttatatcttttgacaaatttgaaccattttcagctattaattgttcaaagttttatcccacaaagaccactttgtcctcttctttccagattacaataatgtgaatgttggatttgttattttttatttgtgcctgagcctctgttcagagacaataaaatcctcctttctctctatagttcagattatgtaggtattcgtgttctgttttcaagttcattgactttttccttagtcttctgcattcgattatggagatcctccaattaagctttttatttcccctaagagttttggttaatacatttttttaattcttaagtttaaattggtgtttatgtattcgaaatatttggtgagactttccaactttccattcacttcacgaatgttatccccgattctaggagcattgttataatatctgctttaatgtatgtgtcagatgattttgacatctgtgtcctctcaatattgttattcgaggattctctttgccatgtgaattaagatctccctgttttttcataatgctgaatattgtggggcttgtaacctggacttctttggattatgtgatgagacactgtgtcttgttgaaatcttaaggataatattgctatttttgtttttgcaggcacacaattgccttgtatttaagctccaagtaccaaccagactttcatgtgttgtcgtttcaaagataactctatttgaaagccttgacactgctgttcagagatctccaaagtgtgtgcaacccagtggtcagtgaggactggaaagtgggccattgcacagttcagctctcaggctctttttaggtaagttgttcgggattagagccacttattcacagctggcaggtgcgtccacaagctcatgaacaactttatggttttgctttctacagtatctgtccaggcacattctagttacttgacacatcttggtttcagtcctctcaccagaaagctggggctgtatttaaccaggtggctctgtcctccacttttcacaattgtctcacatttaggaccaagctgcaggcagaaacagggagaaaagagcagttttatatgtcctttggtttcacagctcctcgaagaaacagaaaattaattacacagtagatctacactatactgaatgccagcaggaagctgtcaccagtcctgtattgttgctgctcctatgtcttgaaccaaagacaccgagagcagtgtcttgctctcagacactgactcgggtttgggtacctaaataataaagcttggagaatgtgggcattgatcccactacctcttgcatgctaagcaagcgctctaccacttgagctaattccccatatcagggaagctttgtttatccttagtgggtggcctggaacacaggtgatttcagggccttcagcgggaaagcagggctctactaagagcagatcttctcattgatggcgcagggcaaggtgcagtggctactcattctctgcaaagaaggaggaaaaaagggaagaaggagaaagtcacaaagggaaaactcacgctgccaaaatgtgaagtttagggtattccaggacagaaaaagacacgtcccagcaaagaagacctatctagacctgcccagctaaagtgtcactgatttttaaaaaataattaaataattaaaaatgattaaatgattgtgtgtgtattgcatgtgtgtgtgtgtgtgtttataaaagtgggatggcattatcacttgttccttgtagctgagactctctgggggttgtgagatggtccagatttctggaaggcacaaaagggattctgaattaatatctgatgaatgaatccactcatttatttgtatttgttatgtgaatgaatgttacaggaatcacctggtgtggagaaaacagatggcaagactatgtgctagggtaaagcaagagctcacgtgtttttgtttttggttttttaatttagaaaaaaaatctgcttttcatatctggttttcctatttaaagctatgtgatttaaggaaaatggtttaactcctctgagctttagtgtcatctacaaaatttggataatgatactgagggaagctgaaaagccatatcaaccaacttatacaaaaaataataaacattcacttccatttctaatgcatggtgctgaaaaagtccttgtatgtggaatattgttcacctttaaggaacctgctctcaagagctgatgcgggactttttttagggcagttctgttgtctctggctgttttgttcatttaattggcacctacaagtctctttgaacattaaaataaaataaagattgtggaggaatagaatacaaacacatagtaaggtgagatttgcataacagagtatagtaaacgatttgtgcctgattctttttgcattctctttgaatcatttttagcctttattctaagtccccaattattgtcatccttttcccaacaagattgtttctctccgccacggacattctggtcagggtctctgcttaaccatcttgacctcctgaacactctgtttgtcctgataacctgatttatgctcaaatgatgctcttccataggacggcttcctgctttgcccaaagagcattcaatttttcaagctgtttagggctccttcctcacccagggtctatttgaaaccttagagggaaggctattctttccaggaagagaaccctgctgggttgtaacctcaatctgtaaatccactggggtaactggggttagctcagttactccagagcttgctctctgagaactggatggtgctgctacttcccataaaggctgaataaaaagaggcatctgcaggcaggagaaagcgctatggtcattgctggaagattccttctgaccattagctatctctctgacctggtgtgagaagggtgacaaaaatcggagacttgaaaacaggccaaaaaaaaaaaaatggattcaaaagaattttaaaagaatcatgcacaagttcttaattagattcttttatccaaatccattttgtctggaaaataataccttactacgtatctgtattctattcctccataatctattttattttattttaatgttcacaagaagctggatgctagctaccaaatgagcaaatcagccacgataacagaactgcactaaaatctctcatcagatattgatacagtcaagaccctcatgagtgcctatgatacaaattcagtgtgagaggccagctttccgcaaggagaaggcaaccaaagcggtagctaatactgagcagttcctattgcccagatccatttctaggtgctgagatccagccagagaatcccacagtcctcatttttcatatgaagaaacatgtgagtgattcaccaccccaatcctcatgtatcatcagttttcaaacaaagccaagtagcctcctgtgcaaaaagctctcctaacccccagttgccttgataggtaaaagtattcttatgacagtgctagaaaaacacgggcacaagtgttccggcaaggtgactagaaggcaaggctaaagttgtcaaggtgacaaagtccctgatggtcctcttgaaagctgaacgtgccacctcatatgtatatgtgtatgtgtggatgcatatgtgtatgttgtgtgtacacacctacacatatatctacaaatgcatgtgtgtatgcatgcatgtgtgtacacgtgcatgcgcacatgtatctgtatacatgtattatgtacacagtatgcatgtgtacatgtatgtgtgtctgtgcatgtgtagatgtatacatgcatgtacacatgcatctacatatgcatgtgtatgcctaaatgtgtgtacaagtgcgtgcatatgtgcactatacatatgtgtacattacgtgtgtgtatgtttctacacgtgtatctgc

SEQ ID NO: 11467 - RNA, 2089 nt, Homo sapiens
  source 1..2089: mol_type = other RNA
ctgaatagctgggactacaggtgcctgccaccactcctggctaattttttgtatttttagtagagacgaagtttcactatattggccaggctgctggtctcgaactcctgacctcgtgatctgcccgcctcggcctcccaaagtgctgggattacaggcatgagccaccacgcccagcccctgcaagcagtttctttaactctgttgggatgccattcgtgggcaaagctagatttgggacaagttgcccagctctgctaggaagagtcagtcctcagggggaagtttcttttcacctccgggatccccagggcttcctgggttgactcaggacttcatacgcagcctggatctccaggaagtgcctctgtgcctcctctgtctggtccaggttgtggtctgggtgccagaccttcactagctcctggtaactccgatgtatttcttcatttgttgccccttctgagaggcccaaaacctggtaagccagctgacgcttctcatcctgaaaactgtgaacaaactcatagagcttcgcccactcctgaaagcagctgctgttgaagccagtctcccccatcagtagcctccagatccggtaaggcagaaggaggacaaactccatgaggcggccaagaagggggaagaagctgaaccaattcaagaaggagccaaaggtttctgccacatagctgagggtggcagctgtgttgcagagggcactgtatgccagtgggcctgtgaaagcaaggtaagccaagcccagacgatagagccgcacactgagcggctctgatgccaccaaagctttgtagcggcgatgcctctgagctgtaatgctggcggccacgctaatgggcagtatggctatggggcggccatagaagataggtgaagtgagaaatgctgaccccagagtgttcttaaagtctgaggtctggttgccaacagcagccaccagcaagacccctaagccaactgccagtgggagggccacaatatagaagttgaccatggaagaaaggctaatcagtgccacaaggccaaaatagatgccaactatcacctgggcagcaaagcgaatgggactcagagggggtgtcacccctctggggctctgcctctgtccctgggctctgttggcctgagctacaaagcttgggagcttccagaactcccagagccagcccagcccacctccccccagggtcagcatccagagcagggcgtggctgtcccttcccaggtacaggtggtggagcccagcagggccccccacagcccagagggcataggtcaccaggagccccttggccatcctctagggcaaaggtctcagaacaagtccggttactcgcagcacagaagtctcggggtcctctgtgagactcatggctgtcatggccccagagttatccttagaccctcaagctgcacgctcctctcttcacgctccgttgaccttcaagactggatggttccacctccaattcccttaaggcagagacatccacggacaggctgcagtgagggacatccaacccaagctgtcctcaaccccccacagggcttgcttgcctcaccggcccacctccgagccttccagttaggggctctgcttctgcacctgagcctgagacctgaggagcctcccaatccagggctgctctgtcccgcgggctatgaaccagagggagaaacgggagcagagggttggagggcaggaggctcgaccaggagggcgaggccgcagcccgaggctcgtggtagtctgccttcctgcgcctctgcgctgcaacggagctgcaatgcaagacgccttcatttcaatgtcccgggctccaatcccgggttctactccgtgaacttggctaagtcatgcagcttcttgggcctcaatttccttctctggcaatctcgtggatctccgaggtcccccagtctggacttgcgggggcttcgggggacggtcggcctcgcgggtgtcacctcccggcagtaggcagagcgcttccctccaaacgccctcagccctcatctcggcctggagaggaaatgctgctctctatatgacctcttagggctcact

SEQ ID NO: 11468 - RNA, 2551 nt, Homo sapiens
  source 1..2551: mol_type = other RNA
ctgaatagctgggactacaggtgcctgccaccactcctggctaattttttgtatttttagtagagacgaagtttcactatattggccaggctgctggtctcgaactcctgacctcgtgatctgcccgcctcggcctcccaaagtgctgggattacaggcatgagccaccacgcccagcccctgcaagcagtttctttaactctgttgggatgccattcgtgggcaaagctagatttgggacaagttgcccagctctgctaggaagagtcagtcctcagggggaagtttcttttcacctccgggatccccagggcttcctgggttgactcaggacttcatacgcagcctggatctccaggaagtgcctctgtgcctcctctgtctggtccaggttgtggtctgggtgccagaccttcactagctcctggtaactccgatgtatttcttcatttgttgccccttctgagaggcccaaaacctggtaagccagctgacgcttctcatcctgaaaactgtgaacaaactcatagagcttcgcccactcctgaaagcagctgctgttgaagccagtctcccccatcagtagcctccagatccggtaaggcagaaggaggacaaactccatgaggcggccaagaagggggaagaagctgaaccaattcaagaaggagccaaaggtttctgccacatagctgagggtggcagctgtgttgcagagggcactgtatgccagtgggcctgtgaaagcaaggtaagccaagcccagacgatagagccgcacactgagcggctctgatgccaccaaagctttgtagcggcgatgcctctgagctgtaatgctggcggccacgctaatgggcagtatggctatggggcggccatagaagataggtgaagtgagaaatgctgaccccagagtgttcttaaagtctgaggtctggttgccaacagcagccaccagcaagacccctaagccaactgccagtgggagggccacaatatagaagttgaccatggaagaaaggctaatcagtgccacaaggccaaaatagatgccaactatcacctgggcagcaaagcgaatgggactcagagggggtgtcacccctctggggctctgcctctgtccctgggctctgttggcctgagctacaaagcttgggagcttccagaactcccagagccagcccagcccacctccccccagggtcagcatccagagcagggcgtggctgtcccttcccaggtacaggtggtggagcccagcagggccccccacagcccagagggcataggtcaccaggagccccttggccatcctctagggcaaaggtctcagaacaagtccggttactcgcagcacagaagtctcggggtcctctgtgagactcatggctgtcatggccccagagttatccttagaccctgggtgccccgctcccagaccgagtcagaccagtcatttcctttgaccacagagtgaaaatggcccgtctcgccctgctcccacttccatccaaatggactttgtcttttgtgtctgttgtgtcacggaagtccggcttccccaggccaggctcctccccagggccctccccggccccctggggatcacattcccgcctgggactcctcccgcccgccctcgcggggaaactcggtgcaaggctctgcagacgcctgcagctccggtgggctcagtgcccagcccgggcccagctcctcccacaccaccgcaccatggccgccaggtggcgctgccgccgatggaagggggggtccgggcggtccccagacaccttgtgcgggtaccgaggcacagcagcacaggactgcccctatggaggggctgcctggcaggagcaagggacgctcctatctgtagtgctcaagctgcacgctcctctcttcacgctccgttgaccttcaagactggatggttccacctccaattcccttaaggcagagacatccacggacaggctgcagtgagggacatccaacccaagctgtcctcaaccccccacagggcttgcttgcctcaccggcccacctccgagccttccagttaggggctctgcttctgcacctgagcctgagacctgaggagcctcccaatccagggctgctctgtcccgcgggctatgaaccagagggagaaacgggagcagagggttggagggcaggaggctcgaccaggagggcgaggccgcagcccgaggctcgtggtagtctgccttcctgcgcctctgcgctgcaacggagctgcaatgcaagacgccttcatttcaatgtcccgggctccaatcccgggttctactccgtgaacttggctaagtcatgcagcttcttgggcctcaatttccttctctggcaatctcgtggatctccgaggtcccccagtctggacttgcgggggcttcgggggacggtcggcctcgcgggtgtcacctcccggcagtaggcagagcgcttccctccaaacgccctcagccctcatctcggcctggagaggaaatgctgctctctatatgacctcttagggctcact

SEQ ID NO: 11469 - RNA, 8959 nt, Homo sapiens
  source 1..8959: mol_type = other RNA
ctgaatagctgggactacaggtgcctgccaccatacccggctaattttttgcatttttagtagagacagggtttcctcatgttagccaggatggtctcgatctcctaacctcatgatctgcccgccttggcctcccaaagtgctgggattacaggtgtgagccaccacgtccagcccaatcatcttatactaaattacttaaataaaaatttattttaacatccttgtgaatatatttaaagaataatttaaaccttaaatagaaatactgtaaatcttgtaaattttccaaattcctgtttttaataaaaagacaggattaccaatataatttccacagatgctttctatgaaggaatataggatatactaaaaccaacacatgatctcaaatacgcaaaaatcaataaaaaggaagactccgttatttcctacaatttaagaaaagtatctaatcctttgagaatttaaaatgttattatcagtttataaaatttaatttacattaattaataaaacctaacatttaatttttaaaatcctggactatttataagaaaaataaagaggaggtctagttgaagttataagatcataatcctcaaactgttccactgaaaggtaatttacatcaacaatttaactttcattttaaaagagactatagttacatatggagtgaaacagttgcaaggctgacctattcccaatcctcttcatgagtcatccatccatgaagctggattaatcatatggtgatccatgtcaattggtaagacaactataatgaatggattagctgggatacagtccatttatcttgctcatagggaaggtgtccagagcaaagagacactcagaaagtgtctaattttagtaagaagtacaaagcacaacaatattattgtaaatgtgaaaaaaaccttactttcccaagttctccacatggccaaggcaggtggaaaagcagtagttatatgcaatcacaatagaaggataaagtgattggaaatccaaaacgagaacagagttgctatagaagcgggattcaggctccataattagaggaacacactgtggggctctcatctgggatctttgctgaacactaggtgtcacaggaatatagttcattggtttagcaatacgcaacatcattgattccacacggtactgtgaaccccttgtcagtacatgtaaaaactgaatgccaaaaagtctagccatctcactggttttcccaatcaggtccagctgttctaacatttggagatttccacggacacggctaacataatgatcaaccattttccatctgtatagatctgtcttgttatcaaaccagtctgacaagactcgaaaggtaaagaggggaaaacgctgatgaagaacatgaaagctcacattttcaaaggtgtagttagttagagccacctcatttctcatgattctccaaagatttagtgtaattcggccaacaatatttatctcactcattgtatatgatccatactcatctctttcagctgcaaatctgttctcaattttgtcatctggcacccgagagatcatccgacataagtcaatacttaaagcggcagccctttgtaagaggtaaccccaggaatgcatctgaatctcatatcctagcagaatatcaggatcatacctctttattatatttgcaatttcatgaaaaagtgccttctcatcagcagcataggtgacttcgagtcctgtaattccagatctaataagtaatggagtctgatatctgatatctcatgtaaagcttttgcctcctgtaagttttgtatgctgactttgaaaccgtaagtattgtttaaagatggtccatcaatctgagaagtttctttctgtggggtatttactgctgcaaattgattctttgcttgtgttaacagtactcttctaagagtgtcagtattacttcctttcttattactcaacttctgtgtttttggttctgttgataatgggctaaggccaggtgcttcaggaagcctttccagaagttttctctgtatgattggtgtactatgaaagcaaagtgattcacatttcccagttcttgccctagtattaattggagatatcactagaggctcttgaggctcactgcaggggcttttttgtataccatcttttattggctttaagaagttctcaaaagccaatgaaggcagctcctctactggtgatgagggtctatcatctccatttaatgctttggaatctggggatattggttgttgccaagggggaattactggagaatcaggggagctataactaatgtaatagttatcatcatcatcttcatctttttcgggatcacttgcagaggcaactggtggcagcatctgactttcacttgcagtttgactacatcccgtggttggtgcttgtaaagcaatctgagaattatcaacatcctccttggtatgtgctgtagtggggagtatacatggacttacatccatttttggaggcactacaggtttgtcatctgggttaactgaagagctaaagttctcagcagattttacaactccagttggcttggttttaggcagtttcttggaacgttcgtattcttctttggcttgaagccacacttgaaccagttgtcgacttggggcacatttgcaaggcataatcacaatttttttatcttcaaccatcttagggctattacttgaccctttattgacaactccttggccactgcgaaggggtgaccctggccttggattctgagtcattgctgagaatgctgttttccaaagacgaagtccttccaaggaaaagtctccctcaaactcagccagatcatttgcaagtcgagtttctaccatgaggagccgtccaccaatctccctgggcttttctggtacatcagaaggattactgcaaaatggttcctggtaaatagtctcagacaggtcatgatccaacaaagttgccataatttcttccctacttgggggggacataagtggtttcagaatgttagcagttcgaggggtgaagctgccatttttagattgtgaaggagagctagtagatcttggtgaactatcaggagttggtgtcaacatatcattgtttcttgaaacatacagttctaaatcttcacaggccacgtctacaagttcaccatcaggggaggagagtattgcagtaaaagaggtattggctgagtcaagagactgtcccatttcttttctggtgtgaccttgaatccagtctgaattgtttggctgtgggaggctaagaaacacttctttgcttactgaactcctattcaatctagatttttcacttagacagtcttctgcctgctgaacacagaaagaatccattattgagttagaccgagttgttagaggatgaaagctatttttccactggttgtggcgacgattctcattgctatctatggttgacttctcaaaaatttcaggacttaaagtaccagatctaatccatgaggctgagtctgtggtatgatgcttgtcttcatcacatttctggttgtcatgacttaaaaactcatttttttctatagcttgtcctggaaaaagatcctgaacagcatcacttaggaacttctgaggcaaattctgatcagctgggacaaactgacttccagaataaaagctacaaaatccagtctgacctattgtgttaatatcaaaattataattatgttcaggagataaactatcttcaagtgagtaacaactttcaaagcctggatctgaaaaaaagatgggactatcatctgatacagagttatccaactggctagagttttgtaaatttaaagagtctactttgagaagtttggggattttttctttttgttttgtacttctgggagttcgaggttttcttggggacgttaccgatcgtgtccgtttatttgctttgttatgctcaagggaaccagaaatatttttatttggttgatgtttattggataatgggtcttgtgtagtatttgcattttgtgctttctgctgtcttttttgtaacaattcttttagaactgccagtccagactgtccttcaccaaatgctgaaggtgttgacacatttcgatttttacactgagaaagtgctttggtttgtgaaattgcttctgataacgacctcggttttactctttcaggtttaaaatttgacatatctaaaataaagcccctttgcttttgctcccatgctatttgtttgattggacttctcaaggaagttacaaagcaattattaggcatttggctttcctctgaagctgtatttcccggagaacaagtttcactgtgctttgactgttccgctatgcacacaatctgctgctgactgtctttgcaatgcaaaaaattaggggtatatgcttggtccagctttgattctagggaattgcgatattcacttaactttccgattgatgacaaatagtttctttgtatattatttgcattatcttctatctttgaggacataccagaagatatctgtgtattctgtgctacctgagataaatgattggaaaggtcaaatatatttttttgaattaacgttgattcctttagagtaaacatagcactttgattatgaggcctttgaacattaatttttgagactccaggtcctatagaattacaaacaactgatggatgcaaatcatctcgtgaactggggaatgtctgcaaatctacagacttcttgctttctaagaaagaagaaaagcagccagataacttctgttgtgcattaattccagtgggtagggaagcagaaaggggatgatctacagcagagcccattagtggcatatctttctgtttaaaaagtagttgagagcctccagaactacttgcaaattcagacacattctggtgtttcagtacaaacttaacctcagcaccagactgagattttattttttcatccttaagtgttgtatgctttctcgatgtacctttctcatttgttttttgttttgctcttggtttcttttttccatcatctactagtttatttgtctgatttcgtttgttccttttcttagtaactatagagggattagcaagctttgcttttgatttcttaatctgtgctcttgcgcgactagtttttcctatacgagaattaacagtcttcttatatacattaggacccttaaaaagcattgcctctttttctgcagcagccatgatttcttcagctcttggatctgtgggagaccagcagcgaggtggagaagaatttatgggacttgtgcttctctcagaaagaaaacctagtttagacataacatcactataattcaggtcacaatcttcggtttcagcattgtaagatggtgagggaggagaaagaatagcatgtgaccgttttttcctgaaagacaaagttcttttaatattttcattatttgtcctttgttgtttaccagtttttttcttagcagatttatgttttgactttcttctgtgacttttctttggtgttagtggataaatgggatatttggttgcaggggagtcgggaacttttggccaaaagtccttcaaaggtgcaagctttttatatagttccattttttcttctgttaatattacttgtttttctttagagtctatttttcctagcttcacaagcatattttttctccctctaaatctattaataataatatactttatgatgacagggggcagctttttagacatttttcttcgttttcgggatttgagagttccatctaaactttcaccaatttccatgggatgaggtagactaatttttgagttgtgagttacaaaacttgactcactgtcttcagtctcataatttaccttgcgtttggctctaagtgtgtatttatttccatatagtccaaaggactgctcagtttctaacgttccatctccaaagtgacagtctataaaaccatctgtgggtgttttattttcaaaagctccacgagtggttttagttaaatcactagccaatgcattatccttctcaggattactattacaaggattattttgtataaaattatcttttgtggatccagtctcactacttttggtagaagtctcctgatgacctgcaagtttccttttattcaattttaaccgggatggtttattgccaggttgtaatttatatgtgacaggagatagtttctgtggtctagtaagacagttagaaagaacaacactgggaaaaaacatatagtgtgctgcttgctggctgaggcttggcttttctgttttatgttcttgaaattcttcatacctaattttaagtttatttagtccactttcatcagcagtgctattaagagaatgcaccatagttctattctcccctgagcatgacagtaattcacaattttcagtaaatgatgaagggaataaactactcagagctgtgctgtttcctttttcatttccttcagaggatactttattttttgaatgatttaagtcagaaaagttgaaagaatttttgcccaatgtattctcgttagggtgacggtgcatatgtataaaaggggaatccttttcgatttttctaatgtttgtatattttctacttggtacttgtcttgtaacagatggaatatcttcttcataatcaaaaatactactttcacaggaagatactgggaggatctctttcttactattctctttatgagaattttctgaatgaacagtactgcttaaagatccagggtatttcatagaataagtgctttcgtttgtaaaagaagtgactgagttatctagacctttttctgtatttttgtttgtctgtgaaaggtcttcaattaaatcttccttgttcaaaacatgggaagaaagggcacttgtgtgtttacactgaaaggtaatcttagcagaagatgagggttctaatgtagcagcatctttgtgaaagatggagggtttaactgaaagcttgcttgttgcaattacagaagagtgggttctagaattttcattgttcaatggattgtcactattttcatctgcagttccatctaactgaggtatagaaagactggctagaagcaaactgttatcactccattccatttcttctcctgaagatgagtcatcatcttcagttgaacttctgtgggtatttctgcacagtgatctctttttggcacaatgttcttcaatattgctgtcccatctctgggacatcaccaaactaagctccatttcctctttttcaatctgtggttcattttcttcatcatcactattttgtggatatttattatttccaaaggagcgacatggtgatggcatcctatttctttccccccgatatccatcactttccaaaccagcaagaagatgtaccagagcctcatcaggactactgtccatgaaaacaggtgactcactcagtctttgggtcaaaggctgaaaagtctgactattttccataaggttcaaaattgcttcttcattaataagagcttcttccactttgtgtctagtgtgacctttgcttgactctttgtctttgtgaacttctaccatattggctggtgtacactgaagcatttcaggagacagaacctcagagtgcaatgttaactcagcagagaactcctgggatccatcgctgtagtccacagatcctgataatgttctgacagagaaatcattctgtttgagaatttcctgaagtctcttctgaaattttttttcactttctgttgctggcacaaacctgtgatcttgtgactcaggttggctcatttgagaagtttcatttctgtttcttcgccgttgcttttcatcttcccatatggcctgtagaccagggtttccaccaatttgagcttcaatgtccagacgatttaagatatcagcagctacagcatccacttctaattcacatgtactctgtggttcaacaccttccaatattaaagagcttggtatttcatcttgttcccaccgaaataaagtatcagcaagagaatttcctgataaatgattcttgcaggatccagttgcatgcaatgtattacttttccttcttgcttttcggaacttgacagcagccagatttattaaattcatgccataaagattgtagtcaatgaagagctgtaggaggtagggaatatgcgcttcatgaggctggtaaaatttattcattatggctccgctttgcaaaagttcacatatccttttcaccattgtaggattgtaaagatagatcttcataaagtgtctttccttctcatgataaccataaaaaggcattcctgatactaatgacactttgaacacatgctgagcagtggaagatggattgcctaaagccacattaagtgctctgtcgatactgaatgccatctgagaaagatagctttctggctgctgtccataaccatcgtatggcacatagaggtaaggaaagatgccatgtagatgaagacatgtcttctgacctgccggggtcgctccgaagactcgcaccaccggcaccttcttgacaggggcctgggtgaggggggattggcaggtatccagcccctgcagcgggctggccatgtagtagtctgcagtcactatccttactgaaaacatgttcgccgccgccgccactgcctcccttcactggcgacccggcagcggcagcagcagcggcggcggctccctccgcagcggcggcggcgccccctccccttctcggcacggccccctcccctcacacagaggcacctcgaggagcggcgggcggggcggtgtaggcgctgctgccgccgcctcctcaggagcacccggcaaggggccgcaggagagaagccctcgagctttcgtcggtgctggtgctgccgccactgccgccaccgccgggaatcacacgggctcctcggtcccag

SEQ ID NO: 11470 - RNA, 2854 nt, Homo sapiens
  source 1..2854: mol_type = other RNA
ctgaatagctgggactacaggtgcctgccaccatgcccagctaattttttgtgtgtgtatttttagtagagacggggtttcactgtgttagccaggatgttctcgatctcctgacctcgtgatccacccacctcagcctcccaaagtgctgggattacaggcgtgagccaccacacctgagctaacttcctggcttttcaatcaaaccatctttgtcacttcctgtccccacctgaagtcagaaagcctgaagagaagatgcctgcctgtcctggctttgcagatggaagccactatagcaccatcactctgccctttccccaaggaaaaagagagtgagaggccaagtgccatggaagatcacttgaggccaggagtccaggaccagcctggtaaacatagtgagacaccatctctacaaaaattaaaaaagtagccaggcatggtggtacatgtctgcagtcgcagctacttgggaagctaaggcaagaggattgcttgaaccccaggagtttgagactgcagtgagttaggattgggccactgtattccagcctgagtgacagtgagaccaacacacacacacacacacacacaatagtggcgggggactgtgggtaggggtgagggggtggggtgggagagcctttcctaacactaacctttcttatttgtaactaccccctctacctggcaggaagaactccaatcaggtgttctcacgatttggccctaacacatctaacctcaaaatcagcattcctaaaatctgccttatccccttaatcttatttctgtatcattattgtacatgtgcttcccaatacttggaatctcctccaccaaaagcaaagtctttcctgtaaatcctcccgagatgctatgttccccacgatactttgcaagtttcactccaactagtcagtaagttcccaaaaagcattctttgaactaccctagcacctatgagggccaggcaatgtatcggcctttcatgtgaccttttaactattaaagtaactccttagaaaacatgtaaaaatcttgtatttaccaaaagtgtaaactgcagaactatatagcaatgaaaacctcccataaagcctgtagatagtttttaagataatttttacttcttttaaaaaattgacattaatattcagtatatatgtacatctcaaaacttcacccaggctgggcgcggtggctcacacctgtaatcccagcactttgggaggccgaggggggcggattacctgaggttaggagtttgagaccagcctggccaacatggtgaaacctcatctctactaaaagtacaaaaattagccaagcgtggtggcacacgcctgtagtcccagctactcgggaggctaaggcaggagaattgcttgagcccaggaggcagaggttgcagtgagccaagactgtgccactgcactccagcctggccaacagagtgagactctgtgtcaaaaaaaacaaaacaaaacaaaacaaaaaacttcaactagactactctgggcacactgtccatggattagccctgctttgcaaggagcagtaaaaaacagaaacaaaacctcccaacttagtgaaaacaaggcattcaatgacagaccagcagcagaaactgcttattacctcctaatcattttatgaagaaatacctatataaaaacaaacactaaagagaacaaatagatttaactaaagtgacaagcataattataaataaataccagattatcagattttaaacaataatctataacagttttactatctaaggattttcactccaagaagaaaaaatacatagtaacgccaagcttgcaggacgatgacttaacagatacattttctcttaatggaaacttatctagcttcagtaatatttctggatgtagcatcaagttgctgttgcacatttttaaaagactggtccagcagtgtttcctcttcatttaaagtattggcaatagcatcattacatggattgtccagaatgtcttcgtttaatccatttgactcctccttttgatcctcatcagtattaacctcttcaaccgtgtgtgccctgggtgtattcattaacatatcatttcctagggtctgactattactcagcagctttgcctgccttctttccaaggccagttgtttatttctctcaattctttgttgttgctcttctgttaggcttctacttaactcagaagcaaacatctcactttcagataagtttgtcagaaagggatctaattcagtagaagtgacatcatgttcattattctccgcaacttcatcattattgctaacaaaatcttcatgtaaaatagggagatcaagtcgaattcgttttaaacaggtctgaacttcctttttacttcccaggtattcaactctgtcaataaaatcctcaaactgcagtttagggaatagcctatgtgcccagtgctccatgtgtctgattagcatcttcaagtcttcagcctctgagcatccagcttgggtatatttcttttaactgttctctttggaggtacacgaacaggtgctccatttcctgactcttcatcaggctcagttccttcaccatcttgtctctctggagaggctggaggtgggaaaggaggaaaagtttcatcttctacatgctcataatctggtaggtcaatcacgccattctcctgtggttctagcatcttttcctcacacagcgacacagacttcttctcagctgggtccacctgcttgcctcggggcgacagagggcgccacggcgtccgcgacggaccccgcccccaggcagtgcgccgcgctcccgtgacgtatttccgcgtcatctgcc

SEQ ID NO: 11471 - RNA, 2798 nt, Homo sapiens
  source 1..2798: mol_type = other RNA
ctgaatagctgggactacaggtgcctgccaccatgcccagctaattttttgtgtgtgtatttttagtagagacggggtttcactgtgttagccaggatgttctcgatctcctgacctcgtgatccacccacctcagcctcccaaagtgctgggattacaggcgtgagccaccacacctgagctaacttcctggcttttcaatcaaaccatctttgtcacttcctgtccccacctgaagtcagaaagcctgaagagaagatgcctgcctgtcctggctttgcagatggaagccactatagcaccatcactctgccctttccccaaggaaaaagagagtgagaggccaagtgccatggaagatcacttgaggccaggagtccaggaccagcctggtaaacatagtgagacaccatctctacaaaaattaaaaaagtagccaggcatggtggtacatgtctgcagtcgcagctacttgggaagctaaggcaagaggattgcttgaaccccaggagtttgagactgcagtgagttaggattgggccactgtattccagcctgagtgacagtgagaccaacacacacacacacacacacacaatagtggcgggggactgtgggtaggggtgagggggtggggtgggagagcctttcctaacactaacctttcttatttgtaactaccccctctacctggcaggaagaactccaatcaggtgttctcacgatttggccctaacacatctaacctcaaaatcagcattcctaaaatctgccttatccccttaatcttatttctgtatcattattgtacatgtgcttcccaatacttggaatctcctccaccaaaagcaaagtctttcctgtaaatcctcccgagatgctatgttccccacgatactttgcaagtttcactccaactagtcagtaagttcccaaaaagcattctttgaactaccctagcacctatgagggccaggcaatgtatcggcctttcatgtgaccttttaactattaaagtaactccttagaaaacatgtaaaaatcttgtatttaccaaaagtgtaaactgcagaactatatagcaatgaaaacctcccataaagcctgtagatagtttttaagataatttttacttcttttaaaaaattgacattaatattcagtatatatgtacatctcaaaacttcacccaggctgggcgcggtggctcacacctgtaatcccagcactttgggaggccgaggggggcggattacctgaggttaggagtttgagaccagcctggccaacatggtgaaacctcatctctactaaaagtacaaaaattagccaagcgtggtggcacacgcctgtagtcccagctactcgggaggctaaggcaggagaattgcttgagcccaggaggcagaggttgcagtgagccaagactgtgccactgcactccagcctggccaacagagtgagactctgtgtcaaaaaaaacaaaacaaaacaaaacaaaaaacttcaactagactactctgggcacactgtccatggattagccctgctttgcaaggagcagtaaaaaacagaaacaaaacctcccaacttagtgaaaacaaggcattcaatgacagaccagcagcagaaactgcttattacctcctaatcattttatgaagaaatacctatataaaaacaaacactaaagagaacaaatagatttaactaaagtgacaagcataattataaataaataccagattatcagattttaaacaataatctataacagttttactatctaaggattttcactccaagaagaaaaaatacatagtaacgccaagcttgcaggacgatgacttaacagatacattttctcttaatggaaacttatctagcttcagtaatatttctggatgtagcatcaagttgctgttgcacatttttaaaagactggtccagcagtgtttcctcttcatttaaagtattggcaatagcatcattacatggattgtccagaatgtcttcgtttaatccatttgactcctccttttgatcctcatcagtattaacctcttcaaccgtgtgtgccctgggtgtattcattaacatatcatttcctagggtctgactattactcagcagctttgcctgccttctttccaaggccagttgtttatttctctcaattctttgttgttgctcttctgttaggcttctacttaactcagaagcaaacatctcactttcagataagtttgtcagaaagggatctaattcagtagaagtgacatcatgttcattattctccgcaacttcatcattattgctaacaaaatcttcatgtaaaatagggagatcaagtcgaattcgttttaaacaggtctgaacttcctttttacttcccaggtattcaactctgtcaataaaatcctcaaactgcagtttagggaatagcctatgtgcccagtgctccatgtgtctgattagcatcttcaagtcttcagcctctgagcatccagcttgggtatatttcttttaactgttctctttggaggtacacgaacaggtgctccatttcctgactcttcatcaggctcagttccttcaccatcttgtctctctggagaggctggaggtgggaaaggaggaaaagtttcatcttctacatgctcataatctggtaggtcaatcacgccattctcctgtggttctagcatcttttcctcgcagaggtggaggccgcgcggcacctggcctggagagctcaccacacagcgacacagacttcttctcagctgggtccacct

SEQ ID NO: 11472 - RNA, 2816 nt, Homo sapiens
  source 1..2816: mol_type = other RNA
ctgaatagctgggactacaggtgcctgccaccatgcccagctaattttttgtgtgtgtatttttagtagagacggggtttcactgtgttagccaggatgttctcgatctcctgacctcgtgatccacccacctcagcctcccaaagtgctgggattacaggcgtgagccaccacacctgagctaacttcctggcttttcaatcaaaccatctttgtcacttcctgtccccacctgaagtcagaaagcctgaagagaagatgcctgcctgtcctggctttgcagatggaagccactatagcaccatcactctgccctttccccaaggaaaaagagagtgagaggccaagtgccatggaagatcacttgaggccaggagtccaggaccagcctggtaaacatagtgagacaccatctctacaaaaattaaaaaagtagccaggcatggtggtacatgtctgcagtcgcagctacttgggaagctaaggcaagaggattgcttgaaccccaggagtttgagactgcagtgagttaggattgggccactgtattccagcctgagtgacagtgagaccaacacacacacacacacacacacaatagtggcgggggactgtgggtaggggtgagggggtggggtgggagagcctttcctaacactaacctttcttatttgtaactaccccctctacctggcaggaagaactccaatcaggtgttctcacgatttggccctaacacatctaacctcaaaatcagcattcctaaaatctgccttatccccttaatcttatttctgtatcattattgtacatgtgcttcccaatacttggaatctcctccaccaaaagcaaagtctttcctgtaaatcctcccgagatgctatgttccccacgatactttgcaagtttcactccaactagtcagtaagttcccaaaaagcattctttgaactaccctagcacctatgagggccaggcaatgtatcggcctttcatgtgaccttttaactattaaagtaactccttagaaaacatgtaaaaatcttgtatttaccaaaagtgtaaactgcagaactatatagcaatgaaaacctcccataaagcctgtagatagtttttaagataatttttacttcttttaaaaaattgacattaatattcagtatatatgtacatctcaaaacttcacccaggctgggcgcggtggctcacacctgtaatcccagcactttgggaggccgaggggggcggattacctgaggttaggagtttgagaccagcctggccaacatggtgaaacctcatctctactaaaagtacaaaaattagccaagcgtggtggcacacgcctgtagtcccagctactcgggaggctaaggcaggagaattgcttgagcccaggaggcagaggttgcagtgagccaagactgtgccactgcactccagcctggccaacagagtgagactctgtgtcaaaaaaaacaaaacaaaacaaaacaaaaaacttcaactagactactctgggcacactgtccatggattagccctgctttgcaaggagcagtaaaaaacagaaacaaaacctcccaacttagtgaaaacaaggcattcaatgacagaccagcagcagaaactgcttattacctcctaatcattttatgaagaaatacctatataaaaacaaacactaaagagaacaaatagatttaactaaagtgacaagcataattataaataaataccagattatcagattttaaacaataatctataacagttttactatctaaggattttcactccaagaagaaaaaatacatagtaacgccaagcttgcaggacgatgacttaacagatacattttctcttaatggaaacttatctagcttcagtaatatttctggatgtagcatcaagttgctgttgcacatttttaaaagactggtccagcagtgtttcctcttcatttaaagtattggcaatagcatcattacatggattgtccagaatgtcttcgtttaatccatttgactcctccttttgatcctcatcagtattaacctcttcaaccgtgtgtgccctgggtgtattcattaacatatcatttcctagggtctgactattactcagcagctttgcctgccttctttccaaggccagttgtttatttctctcaattctttgttgttgctcttctgttaggcttctacttaactcagaagcaaacatctcactttcagataagtttgtcagaaagggatctaattcagtagaagtgacatcatgttcattattctccgcaacttcatcattattgctaacaaaatcttcatgtaaaatagggagatcaagtcgaattcgttttaaacaggtctgaacttcctttttacttcccaggtattcaactctgtcaataaaatcctcaaactgcagtttagggaatagcctatgtgcccagtgctccatgtgtctgattagcatcttcaagtcttcagcctctgagcatccagcttgggtatatttcttttaactgttctctttggaggtacacgaacaggtgctccatttcctgactcttcatcaggctcagttccttcaccatcttgtctctctggagaggctggaggtgggaaaggaggaaaagtttcatcttctacatgctcataatctggtaggtcaatcacgccattctcctgtggttctagcatcttttcctctcacgcagaaaacacgggacacagcgcggacctcggcgtgcagactaagcgcgcttctcgcgatactcgggaactccacacagcgacacagacttcttc

SEQ ID NO: 11473 - RNA, 29996 nt, Homo sapiens
  source 1..29996: mol_type = other RNA
ctgaatagctgggactacaggtgcctgccaccatgcccagctaattttttttttttttttttttgagatggagtcttgcaatgtcacccaggctggagtgcagtggcgcaatctcggctcactgcaacctctgcctcccgggttcatgcgattctcctgcctcagcctcccgagtagctgggattacaggcacacaccaccacacccggctaattttctgcatttttagtacagatggggtttcactatgttggccagactggtctcaaactcgtgacctcatgatccacctgcctcggcctcccaaagtgctgggattacaggcatgagccactgtacccggccccacaatttttttttttttttttttttggagagatgggatcttgctatgttgatcaggctggaaacctgggtcttgaataatggatacatttggaagtgcagagcaaaggccagagagatatccaagccagagagatatccaaggcagaacaaagctcataatttaacaagaaaggtaggcatagataggcctaattatgatgaatgctctcttaccagtataaacaaattacaaagggagtgatgagaagaggcaatgaagtttggggagggaaagaaaagtctgtggtggaggtgataacctgaacttggctttgaggaataaagagttttatatcagggcatcaagagaaggatattcaaggtacttaggaccagaacaggcaaaggcactgaagcaagagagtctggggcaagaatgtctctattgggtcaagactttgacaatattaaagattccattttcttcatatatgcccccctgctgtctttccaataaaggtaagccctgaagcctgacagtcacaggaaaggagagggtgtgtactagagtaacagcacagttgctactcagctgtgaatctcagagcctgcctttattatcttgattattctttggcatctctaggaagatgataagtagtcttcaaagtcagactttactgagaatgagaagggagttctacatgctaagagctccattcacatactaaaagcaaagcttggacaactgaacatgagttttactcctaaccatggataagagaaactgagaatacgatgtgagaagagtctcttcattaggcaggagtggaatgactcccagggcagggagagattgattgagattgcaattgccctgttgggaaataaacggaaacttcaggatgggtatgcgagtcttggagcagcagggttagtcaactactttcctggcatagcctggggaagactgcaagccactcaaaaaagtcctactcatgacttagaggcttacccagtatggcacaggagcactagctcagcattggtggaaggaggtgtctagtcagtctgagaaaatgttggcttcccaaagcttgagcaagatgttcagtacatcccaaagttccaacatcatcccttcccacccactccaaagcccagcagattaacagtcccatagttgggacatggaagctattaaggtagagaccttgagaccaaaggcaatgacagagttgtggtcaggagcagggcatgacagcagtgaacaaaagccagggacccacttacattacccagtagactcagtgacatccagcaaagatggcaggatgagcaccagcagcaggaccgtcaaggacctcagcacatacattagagaaactctttcctgtgtcacctggagatgactgttctcacccactagatgccatcatgaggaagaagctaggaagaacctttgaaaagctgagcatttatccaaagagatggttttaagcctgagataggctatttgaatcgaaagagaacgttatctttgattggcaagtttaaggccatccacctcgtcccacaccttcccaaaaccagatgggatgcatgagaaattgatgtgaaatgaaggaactgtaacttcttttctgcatgatctgagttttaatgtgtgggagctgggaagagggaagaacattgatagaaaatctgaaagcccacagggaatgtggtctaaagcagaggtttaagtcctggctgataatcattttgggttttctgaaaatgcagatcccagtgctccaattccagacctgctaaagcagaatctcacaattgaggccagggaacctacattttagaagctctccttctgactccaatttggaaaccatttatttaaccactagtacaaaaactggccttgaataagacatcacttcctccaagtctgagtacagcacgcaagggcaactgcagcaaatggaggggtgatttagtaaggagggggtgaaaccgaaaatcaacaaggtttgtgtgaactggtctcgacacacttggctgtgaatagcagggatagaaagtagttatggggcttgcaaggacattgtcttaattttcctgttgtcttaacagaggatttactgagcccatgtatgctgtaggaaaaagctagtggtgccagagtttaagttttcagaggaggaataattgacctatgtatgagttctagagaagccttgcagacttacccagggctcagagcacatggcttagtcctgacataaaataccatttttcctctaccacttggctaagaagctgaggaggaactggcagtgagggaggaggttgagaatgaaagttctggagagtcacctaagagacggtaaacacatacctcatgtcttggcttctagagcccggagataagatcagcttcccttgaaaatgttagctcccatgccacatttagtcaagacaacaataacaaaaggctttcttcagggagggcagtggaagtgagtttgagataaaaaggaatttatttatttgcacctatgtattgttcagaagttttaggtcttatgaaaaaaagatttttataaattatacacaattgggtagctttaaaaaataccaaaatatacagtggtcaccctaaaactaacatttttggataatacacttataaattggaaaatgagaaaagatagtctggtataactgcctgaacaacttattaagaacattaacaagtaataacacatattttaatgtaatattgctgactaatttggcacatttaatacacgtccaatatattttctatgtactgtgaaagcttttgggaaaataaagcagcttgtgttacaaaaactgcaacctttcacaaaggttacccacaaaatacttttgcctagccactgcctgtccaacttcagagtggcaccacccttgctattgatctttgtaaccaacgacaattatttcaaaacaattatacaaccctcatttttctttaaaatctttgtcttcctttacttccctgaatacacacgtagtttaccatgacatgggtcttttttttttttttttggagacgtagttttgcactgtcgcccaggctggagtgcagtggcacatctaggctcactgcaacctccacttctcaggttcaagccaatcttctgcctcagcctcccaagtagcgggatcataggcacccaccaatacacccatctaattttttgtatttttagtagagagggggtttcactatgttggccaggctggtctcaaactcctgacctcgtgatcggcccacctcagcctcccaaagtgctgggattacaggcataagccaccgcgcacggcccatgacatgcgtatttctacagcaatgctgtattcccaaatagagttttcttttagagagcctctctctgtgttgacataaatggtgttcagcagtagaacctgaagtaggacacatttcagagagaagtggtgatctcagaatcagtatgcagtactcacaggagccctttgggctctccgcttacatagcttgtctgttctgccccagtgagtcttttctcaggcagagcctcccacttttggcagaggctttttgacttgactttggatttgtcttggttctaagaccactttaataaaggactttacatccctcctgggatgacaaaagactttttgtctttcctggcaagtcctttttgatataaagacaagtgtccctctggtttgagtactctggatttaaaaacaatttttttttagagacagtgtctcactatactgctgaggctggtcttgaactcatgggctcaagcgatcctcctgccttggcctcccaaagtgctgggattacaggcatgggccactgcgcctggctgagtactctggattctgaggcatgccttttctggtaaatttactttgggttcttctgtgtttatattattttttaatctgcatgactgggttaacacttttgggaacactgattttggtttcgtttcgatatggttacatgcatctgtaaatgatttggctcttttcccctgtttctgaacatctcccaagagcaaaaataaacattctaaattttgggcacaggatggctcttttaaagccactagggcaatcgccaccagttaaaacactggtccaaacacctgacttatctgtcaggatttacagaattttctttgctcttaagagattgagaagaaacaaaatggaaattctcaaacattaaggcatgcctgcttttctgggacttcaggtcagctatgtggcttttcctcatgcatgtttttggatcaatgaccatcatagagattgtctatgctttgtctaaactccccaagcttttttattcttagtaccaagagactgcagctatagagttgatatgtagagtcttctaagctctctaattttttttctgcctactttaaatctgctgtttctgccagtgttgagatgaaactcactccttacggcattccagccaagaacaaaaagaaaaaaaaaggtcttaaagggccttaaattaatggctttataaattataatagttccctggcaaccaacacctagaattaagaagtatcccttttaatgtaaatttaggtttgcctaataactgcttagggtgatggaacagttaattaaaggattaatagcctaaaagaactagataaatacgtataaaaattaggctctcaaacaggtcaaaatcttgagctcagggcaataatataaggtatctctggtatagcataaaaattgcttgcctgctatgcaaaggctaaaagaacaaaacaaaaacccctcatccacaactgctaaaatgcttccctgcctgcactgactagtcaaaaaaaccagaatggcaaacaaaagatttgttactaaaaattcaaggccacctggagattgttttttcttatacaattcagccagtcctagctaaaaatgtaagcatttaaatattaacattaaactcatttgaaactgaaaaaagggaaaaaaggggttggggaggtggggtaagaggttttttaaaaatccaaactgctatttaccaaaacttttggttcacagctttcataagattacctattctgcatgtttacccagctgagcaggtcccactttctcagaaatataatttgaatccaataactgtcttttataaaccagcaagcctgtattactatcgtatgactaaaattctaaaatgaaagctatgtttgtgtatgtgtatgtttaggtgtgtttacacatatgtatatatatgttgtatgttgtgtctacgtggtaaaatctggcagttggccacaaatcccttaaggaattctattcatcaaataaatgagtgctaatacaaaatatatagtaattaacacaagtgccttttagttaatataacttaaacatctgataagctggttttaaaataattggtaaatcaaaaataagtgtctttaaaatttttgcctgaatttactactcagttttatatttgtctctgttagactttttaaggtcataaaactataaactcaacttaaaaacagaatgatctttgtataactgtaagttgaactaattttgtattattgacttcagctgtgtcctctgagttactggcaaaatacctacatatttcatttttatggttcttaattgaacacatgatactcacaggtaataaaaatggttaacaggaaaataacttgaaatgactagctatgtctaatatctcagtttttataagtaatctaggaataattgttaaaaatgaattgggggccaggtgcagtggctcacgcctgtaatcctagcactttgggaggccaaggcgggcagatcacgaggtcaggagatcgagatcacggtgaaacctcgtctctactaaaaatacaaaaaattggctgggcgcggtggcgggcgcctgtagtcccagctactcgggaggctgaggcaggagaatggcatgaacccagaaggcggagcttgcagtgagccgagatcacgccactgcactccagcctgggtgacagagcgagactccgtctcaaaaaaaaaaaaaaaaaaaagaattggatggattataaacgggataagcaagggtgagacatggtggtatgcaggtatgcatctatagttccagctactcaggaaacggaggcaggaggattgtgtgagttggagtttgaggctgcagtgtgctacaattgtgcctgtgaacagccactgaactccagcctgggtaacacagcaagacattgtctctaaaaaataaaccaaaagaatgtttttaaaaataggatgttaatgaacttttcatgtaatttgaaatcttataaattaatcttcagtaaatgtctggatcatttccaaaaaaaaacaataaactgctgaaaatattagtttgttcttggcttcctaaattatagaaagactaaatatatttgggcctattaatatacaaagttataaggaaacatgtttctaaaaattataatatggttctcatttataaaatgctgatataacacttcaaaattttgcttcctaggttttcactaaaaattaaggttaataagttaaaatttgaaaatacacaattccatatacaaagtgtacccaaaaaaagatgttttgatgagaaaagttataaggcataaaaattgctttttattgggaaaaaagttgtttaaattcagagtttattagaggttgtttcaaatatggaaacaagacagaaaggaaccactaagtaggaggaggagagaaatatgaaggaagttaatgggtgtgagaatgtacctttggtaaggaaggttacaaaattaacagaataattctgtatgagtcttgcatagtaactttttatcctaaagcaggatgaccagttgtttaaggggaagtataaaacaaagcagaaagtttaagcatgtcactgaaggtctgtgcagatcatgaaatgttcatgaaggatacatttatgaaaggagttgtgtgtaatgaagttggcaataggtcagaatgaaatcataagacattgagcttacatatatacttgtacatatgtatatgtacaataatacagtatattctatacatatgctatatatttgtatatacacgatagtgtaaatgctatacatgcactatacacacacacacacacacacacacacacacacacacacacacacaaaatttggtccccaatgttagaacaaggttctttttaaggatctggtcttaataaaattgaaagaggttttaatttttaattctaaaatcagccatcttctaaaccacagtttaaatttctgccatatttccttctgagatccgtttaatttcccctagattcaggttagaaaggctgtcttttttcatttaagatggtcatttcatttcttgaggtagagttttcttcttgaagatcctgatttatatctcacaagttcaacctttgctgtatcttgctgcaccttatttgtaggtcacacatcattgcctttagctctttctccccttaagaaggtacatctttttgtttggcaggggtgataactcttaactttttcattagctcctgtaacttttttcctctggttctaactcttgctgttataacttgatactgaaatgttctgtagaaggcctagaaaagcaatgttttcctccagtataacttgattctgaattcttggctcttctcatgtttgaattgttccacgcaagcaggaaatttctcgtaatttttccaagagccatgtattctgttcaacatactagctttcttatttacattcctctataaggcgtacactcataaccttggaaatactcttcctgtgtctgattaaattcaagtaccttttcatcagattcaactttcagtatatccaaataggcttcccataagtaaaggcagtcacactgcaagagatttttctttaccattttggcaactggcctaagaaaaattttatgttctatcaagataaattcttgtgtttaagttttttttttgcttgggaaaaatgaagctttgaaaagatggtttttaaatgtatgtaactttctgcattgcttcttaagtcttttgattatcattcttgttaaatattttatagtgacctgtgatcctgtttcgaacttttgacatctttgacaggcttctctaggctcaagttctaaattaagtgtttttgacttaaaattacctttgagttttccacttgggcctctggaaagcctcagagcatgtgtatgccatctggtagagatgttagctaattaggcttctttgatgtattaaattgtatgaaaagcattgtctaatgatgtaatactagacacagttacatttatgagtatgttattgatatgagtgttccaaaattgtacgatgccgttagaaatatgtcatcagtcataattctgattatgctgtttgccacaaaaataaccaaaactctttgtctatttctggttatggtaaactctcatcagatttttaatcatggttattctaagtttttgtaattcccagttattgctttttctctaaaagcatttgcaatcagattcatggaaaagatgctaacacacttttaaatacaggttactaatcactttaataccaatggactaaatattttttcagaacttcaagaaactgatgagtccatgtaactactaattaagatcaaccacaacaaaaaaagttacatgagactaagtaactgaagatgtgtctgtgacttttatttgaagcattattgtttttttacttaaatgttttgttttccatatttaaagaaattctctcatgctatctatagtttacagcaatttggaatacttttgtgaacaaaggtagaaatatttgcttttcctttcttcttgatccctccaatttggaaactattttgagtattcatttgtttttgtttttgagacggagtctcgctctgttgccccagctggaatgcagtggcacgatcttgtttcagtgcaacttctgcctccagggttcaagcaattctgtctcagcctcccaagtagctgggactacaggcatgcaccaccacacccagctaatttttgtattttttagtagagacggtggccggggggaggtttcactatgttggccaggctggtttcaaactcctgacctcaggtgttccacctgtcttggcctcccaaagagctgggattacaggcatgagccactgtgcccagcctatttgtgagtactcttaaggcaatatgatttgcctaagttcaataaaaatcggctctcgttataacaggatacaattggaaacactggttgtattaccaaggctttgattaaaatgtcatatttgagaatgtgtagaatgcctggcttcaatggttctcagcattacactgaattaaaaattatcatttcctggcaggcccaggaaccttaaaactataggtaaaatctaaagtctaccttgacttagcttcttagcctcaaggaggtttttaaatctgagattactgtgaccatactactattcttgcagacaaaatctgataaagtttacaaatctgttttattctgaacatctttggtaaaaatcagggtaactttaagtttctgaagaaagctatatgtacctgttattagatcacagctctgtaccgttttgaaactcctgttatccacctgcagactggatttgctcctgaatcctcctaatttccttcaatatttggctatgactctctaagaaaaaaaactactcccatgctctgaggcctataagctaagatgtgattaatttttaaaggagcaagtctcatgctgatgtatgggtcacacaaaagttcaccataccaaccaatgccatagctagagacattcaaactgcaaaccaggacaaaaagttgatgatttcaggctgtagacatttttcctaagacatcagagcaagaattgtattacaatttgatttattcaattggttgcctgtaagcctaggttcagggctcaaaaccattatgcaaactgggattgtcacattactattaattttgtgtatttcctttttaaactttgtatctgttatttgccaaattttctgcagaaagaagtacaattcctaacagaataatgctagcccagcactttgaggggacaacaaaggactaaggaaaaaaaattggacttaataatagactccaggtggacttagcctaagtgccactcccttaaagcctccctgccctcaaaggtggctaaaagggttttaacactgacttttagttgccaatcactcctgccaatgcaggatgcaggaccagaccaataacccgggaaaggtctattctgtcaccaagggacaatcaaagcctaactacaagatgattcatcatagatactttcggaaaaacatcttcatcaagagagggaaaggtgaaagctgtcagaatcaagagtcatgtttccaaaagccctgacaaatggagccagggaagtccatgaagagagggattttacgcactacctcaaagacccagaagaaaccacgccagcttgcacaaacactattcgcaaccttacacagaaaatacttttgggacatctgcctagaagccgattgtccaaacccgaactggcagcatccttgttattaatccttgtagccaagaataattatttcaagacaattatataatctttatctgtcctttaaaaacctgtcttcctttaccttcctgaatacacacagtttactatggcatgcatattgccttcacaatgccctattcccaaataaacatcattttcttttagaaagcctctgttatttaggttgacagttattacacctgaaaactaaattctagctgatcaataaaattctttggttctactgtatacttttatttggggatatctgcttccaaacacactaaagtacagtatactcaattttaaatatagacagtatatttaaaaaaaacataaaaagtatgtcgaacatttttaatttcaaacaccaaacttaaatagactaataacacagatcttctgtggtccacaaatcatggcaaaaaactttgttttcatatgcccattatggcttgctgactggcttactgcattttagattttccttatgattttagtagctttctctaatggaatgtgctgtgagtgaagcttcaaacattttccattgaatatacacagacatacaaataaagactggaaaaaatatacaccagtcgttttctctggttgttggaatctgggtgattttttaaagtcccatccactgggctgccagtaaaagaccacaaaatatttttgtgtatttacaggaacgtgataatcaaaagttgttgtgggaccattcaagatgagcgtggggaagggaagcccatttaaacatatattcaaggaaaaatatattaagttacctgaacatttgggtagaaatactgagcactgctatggtctgtctcccaaactgtccctcaaatgtatgatgagattttatcttcattgtggtggtgttgagagctggggcctagtgggagatgtttggttcactgaggcagatgcttcatgaatggcttggtgctgctcttgcaatgagttctcactctctcaagactagattagtccccaggagtgggttgttaaaaagagacttgtttggttgttgtgaacaagtgggttgtttgcacgtctgcttcccctctgaccttctccatcaagctatgaagcagcagcaaagcccttgccaaaagccagggccatgcccttgaacttcccagcctgtagaactgtgagcatccttcataagtgaccctgcctcagctatcctgttatagtaacacaaaacagactaagacaggcacacaaaagctgaggactgctgtcgactccactttcaagggctaccaagcacagccacatcaccaaagagaacaattcctgacctccttggaagcagaaacttgactctccgggcaagataactgttgtctttttaaaatttcagtgtcaaagttaaaacatgccttgatcagtcaaccaaattactgctaaaccagtattgggaagcttcctaaagcactccaagctcctaaaaacaggcagcatgaagtaaagcagatagcatctttgcatttaagaagtcccagaaaggttttggaaatggcattaatgtaaatgttcacattaagagaaaacggtttccctgaattgagtgattctttctactttctagtgctgtacaggataggctcagcgtttggagagtgttaacttccagtcatgtgataatggccaggagcaaccacaatgattaacctttagatagaaaacacaatcctttgcttttgtcttccttatgtatattagattaggcttctactcaatgctctgtaagttaaaacatttcaaaccaaataggccactctattaagtcccagcttgagcattcttcagcttctccacattttccattgtttgctggcaaaccagtacagtaacctgttaaatacaaagcaagggtgtggtagattgactgcatttaaggctccaattcttcacccctcctatgttctctcccttggtctaataactctgtagtgcctttccacactgggtttagccatgtggcttgtttctggtgaatgctagttagcatgaagcatgcagacatgaaagggagttatgggattgggcttggctgttgttgccttctacaacctccacaaaaacatgcttgtttaatggaggataggaggcatgtggaaaaatgccaagtccttccaggtgaggccaactccctcatgaacgaggaaagactacaactgctccagagacatctagccgaaatcacttatctaattcataaactgtttattgctgcacaccactgggtttttgtggttgctacgagttacttttgcggcaataattgctccaatatgttctatgtgacatttctgagtttaacatcacatttacaaactttcttagagaaagatttgttattagcaaagaccttcagagtaacctttgcctggtattctagactgtgcagatttagccatctaatactgagtacccacttcaggctgaatgatctctcaagtgctctcatttagttctcataaccaccctaaaaactaacttcctcattttagggaactggaggaaatgaagaactttaaggtagactgatgaaaagatttatctaaagtcacataaattggcacaatcagggtccaaaccccaggcctccgattctgagtcaaactgcattttccattacatcggaaatgaccaaggattaaaattagcagaatgttattctgtccagccattaaaatccaaaaaaaaaatttgttcaaagtaggcaattgagttttcattctattatccaaggtaactgaagtatttgactgtacaggactgcttccttcaagtgttccatccttagcattcttgttaaaaatggcctttaagatattgctattcccagtcaagaaatacccagacaactaaagagactaaaatcatgtaaatcatccatttcccagttgaatcttaaaaaaaaatttatgctcaatacctctctccagccaatcactatgtaaattgtgaattaagacattattacttggtggcaataacggttagaaaaaaagcacatccctctccctctcccgtctccccccgtctcccactttctacggtctcccactttccaccgtctccctctgatgccgagccaaggctggactgtactgccgccatctcggctcactgcaacctccctgcctgattctcctgcctcagcctgccgagtgcctgggattgcagacgcgcgccgccacgcctgactggtttttgtattttttggtggagacggggtttcgccgtgttggccaggctggtctccagctcctgaccgcgcatgatctgcccgcctgggcctcccgaggtgctgggattgcagatggagtctcgctcactcagtgctcaatgttgcccaggctggagtgcagtggcacgatctcggctcgctacaacctccacctcccagccgcctgccttggcctcccaaagtgcggagattgcagcctctgcccggccgccaccccgtctgggaagtgaggagcatctctgcctggctgcccatcgtctgggatgtgaggagcccctcagcccggccgcccagtctgggaagtgaggagcgcctcttcccggccgcccatcgtctgagatgtggggagcgcctctgccccgccgccccgtctgggatgtgaggagtgtctctgcccgaccgccaccccgtctgggaggtgaggagcgtctctgcccggccgccccgtctgagaagtgaggagcccctccgcccagcaaccaccccgtccgggaagtaaggagcgtctccgcccagcagccgccccgtctgggagggaggtggggggcagcccctgctcggccagccgccccgtccgggaggtggggggcaacccccgcccggccagctgccccgttcgggaggtggggggcagcccccggccagcatccaccccgtccgggaggtgggggggcgcctctgcccagccgccccgtctgggaagtgaggagcccctctgcccggccgccaccctgtctgggaggtgtacccaacagctcattgagagcgggccatgatgacgatggcggttttgtcgaatagaaaagggggaaatgtggggaaaggaaagagagatcagattgttgctgtgtctgtgtagaaagaagtagacataggagactccattttgttctgtactaggaaaaattcttctgccttgggatgctgttaatctataaccttacccccaaccccgtgctctctgaaacatgtgctgtgtccactcagggttaaatggattaagggcggtgcaagatgtgctttgttaaacagatgcttgaaggcagcatgctcgttaagagtcatcaccactccttaatctcaagtacccagggacacaaacactgcagaaggccgcagggtcctctgcctaggaaaaccagagacccttgttcacatgtttatctgctgaccttccctccactattgtcctatgaccctgccacatccccctctccgagaaacacccaagaatgatcaataaatactaaaaaaaaaaaaaaaaaaaaaaaaaaagactttagttcaagttgagaccaaagactgtgctattatggggtggagaaaagtatcacaattttggtaatactaggcaagatgtaacctcaagtctccaggcagccccatgagcttccctgtgaatgagaacagaaaaagttcaggagccaccagaggatgttaaggaggcttcctagagaagacgtggcaatgcacctgatggagacgtttaatttcttcactacaaggaatttcaaacttatctaaaaggaaatagaatacaacaaagctcccttacccaatcccaacaaacaaccatcaatgtcctattcattcatacctccatctacttcctctgtcacatactattttgaagcaagtcttacccattgtattttacccataaatgtttcattctgtatctctaaaacattgtctctagacctcagcaaaaaaaaaaaagcacatccacttttacaatggtcacatacaaatggggaaagagtggatataaaaaatatgcacccaccttcaatcaaatgcgatcttttaaagaatataaacaagccagattcttaggtatctctcccttttgtaattttgattctgaaaaaatatttaaagtaatcaattaggtattctaaaagaaggcagttttctaggggtttatttaattataggggggttggggtagagagattaaaaacgggaagcagtgcataggcagtatgaagtagacactttggcaaataaaaactgcaccgtatgacatgtcacatagaaattgttagagactttgaatcctaaaatttagtttaccaaatgtagctttttatgttttatgttttaccaacaaataatttgtatgttaaatttaagcatctgaattccgaaatgataaagaacaggaaaataatgactaagctaacaaccaaactttcagagtataaaattttgtcagtggttttcattttagaattaaaaatttgaatttccctttgcctacaagtctaagtaacttgcagcagcaaattcccccactgacaacttcaaagcatagcaagaatccacagtggtttgcaggccactaattcttttacagatgaaagcattcaattatctctataaaattcaattccttagaatatgtgtttgtgattgacgatgtacatttttaaatgtggtgataacacgttattattcatgatttaaaagttgaaatgaagtagcttgtggttcttgggtaaaacagacactaataagttttttttcaatataaaagagcaacctagacattcctataaaacatttttattccaggtggtaagctggcttaaattttcacttttcagccaggcatgatggctcacgcctgtaattccagcactttgggaggccgaggcaggcaaatcatctgaggtcaggagttcaagaccagcctggcaaacatggtgaaaccctgtctccactaaaaatacaaaaagtagttgggcgtggtggtgtgtgcctgtaatcccagctactcaggaggctaaggcaggagaatcacttgaacccaggaggcgaggctgcagtgagccgagatcgccccactgcaccccagcctgggcaacagagcaagactctgtctccaaaaaaaaaaaaaaaaaattcgtttttctcacagcagcacatttctaaatggcaaaccatttagaagtgagtcatcatttgtattaaaatcttatttacatggtacttatgtagtttgatcaaatactgccacaatatagtttagaggcaagacctctcatgaagaaaaactttacaagatttaaaatcagagcaaatgaatttcttaagttcaagatacgtactctcaatggagaatcgctgttgggcagtggttaaggcctctgatttgctacttattagaaaaatccacatatatacaaaactctgctaaaattccaatggcttctctagatgaatcatctttggctgtgagcaaaaaagttaactaagtttcacttaatacacacacacacactagggtttatatgtagcaacttcctcatcctcattccacaggtagcccgttcttggctgggttatggcttgtaatctcagaaccactgcccccaaatgactgctcagaagcacaatctcactgcaaactatggaacccaaactatacagctatccttggcttttaactccaagctatctaggccttgtgattatatgtgggcttcatagcagaacctaccaggcttgtggttatcaattttctgctcaccatataagcagtagctcaataacaccgtccagttttcatgtatatccagacacacaggtgagagttctgttccaagatctcattttgaccttcttcaaaggtcttctccatctctccaaattgaatgtattcttcaaccctgggcttactgtattctgcccatcttcttcctggaccaaactgttcagaagttaacttctttttcctgtcatcacatctctttcctaaactactttagaacttaaataattttattttcacataacatttagaaaggtgcagaggcagccaacaaaactattgaagacagactgtaaaaactggcaaatccccatctcaaattccatttattctataaccaataaagtcatgcagtttggacgggagcacagtaatacattctgttctcatgtagcttcctaagtatgcttagtctattgttcatttatcactgaatctgttatctgctaagtctgattcaatgttcttgccttctattaatgtgattttaagaattactgcatgtctcactatggcaaaatagcatgacatttgttttacaaaatcagttaaaccaattctacaaatatttccatacctatttattgcagcaaaagataatttttatgtgtaaattagctttttgggtttttctattcctttatttgtaaacttataatttttaggttgggcttactattttgatgagaagggtgaatctgtcaaagggtaagctggataactgtatgttgcaaacatgttcctgaacattcttcacccaaacttagacaaacctggagcttaaaataattacattggatgacatcagtttgatactgatgcctgcttcctgcactaagaggctttcaatctattttgaagagggaaaaacagaatatgccaagtggggagacagcccaaacatagaccttaatacttctctcatactcttcagccatttgatgaacatgtggaattatggatgctagggccattataaaaatctcctgatacagaacagtgtcactacttcaagctaagcagtgacaggcaaagccaggctgaggtgacaatgtagaaggatctcgagtcagccctcaatgttgttgttcaatgttgggaagtcccttttagattatttatacagtggcaggtggtagcaattacagtaaattttcttgggtttcttcctaataaaaaagtgttgataaaactacaccagtcccaaggctattcaatgccacgtaaaatagtgtattttagcatttgaggtccctttttgttgcatactaaagcatgtttaaaatggtttgcagaaaacagtctgctaaccagtactgattcatccacagaactgaattcttgcaaggcacaaaggaagtgtggctgacctaaatatttctcatttttaaaattattcatactgattatatgagattatatcttatctagtatttttcaatggagccttaaaaatgttattttgttaaaagtatatttcagcaaatttcaactttgaagatgtttttgtttacagcatagatcttatgtattagagcgctaatgtagcataggcaaactctgaaataaataaaaatgtataaatagcactgtgcagtgtgtggtgtgcgcctgttgtggggttatattaagtagtataaatttatctcccggggggataggataatcttttatgtaacaccaaattaaaaaaacaaaaacatgtactcttaaaatcatatgtccatatgtgaaatacaatcactttttttggtttccatataatttagggagtgaacaccaaaatgtaatcccatataaaaaaagatcagtttaaataaaaattaaaacaattaaaaattagtcccatagtaacatggtaaacaactcaaatggctttcttttaatgctaggaaaactgtccacctttcaacggtgacagggctgttaacacaggtaagagcaaacaaggtaaaaagtgaaagcacatacagatgatgcacacaaatatatataaaaattgaccagaaatcacaggacatgtaagcaatgttttcttaagcagaactttttttgtactttaaatagactaaaatatttggtgtaggtgggagaaagacatcagtattcaacaattttaacttgaaaaccagctgtaataaagcctcagctcattgtttaataaaaataaaaaaggaaccacatcgtacttttgacaatcatagaacgaaagctcacaaagaacacatttaatatctccatcacagtgcaccaaggatgcagccactaaggacttccagagggaaacaagaacagggtctgcatccatcatattgcattacaaagttaatgccatcagagaaaaaaaatctcacctcacgtgctcaatgttctagctggtaagcaccttatgagtatgaggctacaattgagagaaactgctcagtctgcatcaggacacccaattccttcacttgccattggctgatgcatttaatcattttaacacaacattcacggaaaaatgttaacaacacattctggcttctcgagcagaacagactgggaaatgcagtagacgccagagcatcaaaggccatgtatttcctcacaagaaaagaaatctgcaacaattggtttccttttactatgaaaaatgtaaatttcagattaagtttaaccccataaggacgcatgatttgtacttacatatacacataggttcagaagaacttagctatctagttggcctcttctctgttccattataacatcagttaccttagctggatcactaagtgtgagtctcaccaccatactggtaccttcagctattacctgtgttataaatctcatgttccattcaaagtactaaatgactggatggcacatatcccaataagtatcagaaatgttgacagccatagtgcagctgagtttagaagcaactatgacaacatagggaagtaaggataaatcacaagaacacctaaggtggtcagctccttctggtgtgcctgggacttgttttgagtttagcaaaaactttacaagattaaaaatcagagcaaatgaatttcttaagttcaagatatgtactctcaatggagaatcgcttttgggcagtggttaaggcctctgatgtgctacttatcagaaaaatccacatatatacaaaactctgctaaaagttttgtatccagggaaagtcccgcatccagggaaaccctcaatcccaggcactttagggcagctggtcaccctgagaacactacccactcgttccttaatatcactagagaaaaggtaagaactttcaagggcataacctttaagggcatcagtccccaaaatatttttacatcactagctaatggctagttcctctaagcttgctaaaaggctaggaagtccagaaataccttaaacgtgttaactttaagaagagttggtagtaatcaagcaaattagtgagcagtgtataaaagctcactcttgaaatctgttttcagacaaatcttctaaaggttcttctagctttgtccagttatatggtattttactgtattctctttttgcaattaatccagttttgtatgtcttttctttcttttttaggtgaaaatattctatgccaactgttttccacagtcctgcattatatattaaaacaaaggctgccagctggagacacagccctccgattacaaaggcccagaatgttacttttaactgtgctccaccaggaggtctggccttgggaaaagatggcgaaaggaatattctcagatatgaacattttttattctgcctacaatgctgtgatctagttcaacaactgcagaactgttctcatcttaatcgctgtagtttttctttctttactcttttgtataaaaggttagtgtcacagcttcactatcactaataaaaagatacaaatatgcctttcaagtcagggttggaaaagcaaaactgaggtgtgaggttacactggtctaagaaagtaccaatttgggttctatattttgtcaaacagttgggtttttaaaaaaattcaaaactcatgcatgttacctacttgtcatgtgtgaattatttctcacaattttaattaatctgtgtgtatattagttatataaagcaatggatttccacattcttaaagcaggaacctatattcaccagaaaaggatcctcctgtttctcatcaaattttttttcagctcgaacaatccaagattgggaatagtaagagtggcaaacaaatgttttcttagggacttactgagaaaagaaaaaacttactgggagaacagagacttagtaaaatttctattgctacagacaaatgctaaaaaccagctttataataacagcattataaaggatagaacttaatatagaaccagaaatatggcaagttacctagtgattaacattgtaaaatagtcaaaaactttaaagccacagagaaaggaaaacaattatgaaatggaaaatatataatatttaagtacttttataattctaaaacttcacttttgtccttaaatcaatatattacggatttcattgttcaataaattaccatctttaattaaaaataagtaaatcaaagagcatatttggagaaactaagagctgttaactgtttggagggtaaaagaatacttttctcgaaatttttttgaagaaaaatctaaaagccctctatgttgagttaatacaccttctgacccccatcatcagtggcattattcttccaagggactcttatatctaagcaatggtgaagttctggattcattatggatctcatggcaccaaaccaactggcactgaagttaagttaatatactccagcgagatcacctgtgggtcaaggatggcccagagaatcttggaaaatccatttatattgagcaaagatctgaatcaccttcaatcaggctgtaagatactagaaaatttgaccttgtagtagtatttcccagggtaacttaagcagcaaccttgcaccagaagaagaattaaagagggagcaatctagtattatcaacaacaacaaagttaaccctaagttagtacatcccagaatctgctggatgtataataatttagtaacggggtatatggcagagctttctttgatgttaacaaattttggctgtgattcttagttaccaagttgccaaaaaatggtatattaaatgaactgccaaatggcagattaagaaaattaatgtactccaatggtctgtccatgaaaggaaaatgtacacagacaaattaagaacattttaccaggatctgagatttaaacaatggaacaattgttttaactgttagaatgaccccaactgttaagtttgtctatgagtgtatatgtatatataaattcatacacatatattatttatttccttcttaaaaagactgaggcagttctgctatatatagttagctacaatattcaagataaaacagttcctactcaaaaaattacatgaacacacgagataagttcttatcgtaaatgctatcatgaggctatctagtatagctcatatttcctggttgtaaggctcaaaacacaggaattccactccaagagataatttgcccctcaatccctacaaagtgtagtctaaacaaacaaaatggtaataaaaaattgaaaaggaagatataaaaagaactcaatagcaggattctgactacctctggagaccacacactatcattattctgactgtcttaaatacaacaatccaatatgccccaagatggaaatctggtatcgtagggaaaacattggctgcaactgtcagaaaagttcataatcttaaacataatttatgccatttgccagtcacaaagacatttactgaacagaatttttgagccatttgtaaaattaaaatgattgatcaatttgaatagcaaccttcatgatgaagaaattaggactctaggtatgaaaagcatgttccttttttgttaataagttcaaaggagagaaacattctgatatatgcagataaaaatatggctaggctgggcgcggtggctcatgcctgtaatcccagcactttgggaagccgaggtggacagatcacgaggtcaggagatcgagaccatcctggccaacacggtgaaaccccgtctctactaaaaatacaaaaaattagccgagtgtggtggtgggcgcctgtagtcccagctacttgggaggctgaggcagaagcatggcgtgaacccgggaggcggagcttgcagtgaaccaagatcgcaccactgcactccaggttgggcaacagagcgagactccctctcaaaaaaaaaaaaaaaaaacaaaaaacaaggctaacaagaaagaggataaccagcaagtaccacctggatgtgtgttgtcaggtagaaaggaagaataaaattcaggcaatgaatataatagatttagcaaagtaaagcatatgaaaggaagaaatgtttgatatgtctaagtatcaatgccttcgatcagagtaagaaaaaagtattcattgttcatgtccacagactagatatctaaagagatacttggtgggcaggggcttgggagggaaggcgcaaattggaatgttcagcttttaaagtaaagactgtacatgaagacatattttatgtacagtgaagattgtcttgtgttactttatatcccaacataaacctacgccaccctcagacgaagagggtatctaacactgaataaatgctgaacctatttagtagttaaagaaaaaagagaaggatcttaaaggtatatatgggaagcttttaagaggtagagaaaccaactgggtatatattttcttttatttgatttcaactagcaagagactaagactgatgtttgtttgtttgttttaccttcaaagtcttagtcttaaattgacaagggcacaaaaaaagtgaaattaaaataattttaacaaaagggaaagcatttgacagtgtttaaaagacagacaaatcaagcaaaactcaatgtggcttaaggtaaaaaatacaactaggtattaaacaatttgtaaaaacttacaaagaaaatttagctttcaagaaaaattaggcagatttccttctgccaaagtgacaggtcctgaggaaaaaaaacacaacctctacaagaccaagcacagctcaagggtcagggccccgtcctagtcatctttttattattcaatatccatcacagtggctgggcaaacaacaggcatcaataaatgtttactaactgaatgtgtattataaggtataatcggtataactgatatagctcaaatctaatcatgaaagcttctttaaagtaggataaaaagagcacaatcagcggtattccagaaggtaggcctaaatccagttatatttttctaatcgttgaccagtggttataaagactttctgagcttctttttaaagcaatgaaactctttccaaaagaaaccccatgcagttcttcagtacagaataaatatgccactaagtcagtgagaactccaacagcctcccctaagccagcccccaaggtgtctctgtggaacctactggaaaaaatattactcatcttagaaatgtgatagaaagcatggccattcggttctcaggtcatcattcctagaaaattaacagtattgtgaagaataaatcctaagtaatgttgctaatttaaataaagacaaaaattcaacaaagaggggattctatcacttagaaaaatgaaaaccacacctataaatggggggaggggcagaaaacaaaaaaaaaatcaggccacagtagataaaatacaaaaaacatcatctcgttaaaaagcatcaaacacattcacacaaatgtaattacaaccaggaagtaaactgctcaacaggtataactgctcaataggtgttttcaaagagttgagtcccaatttcatactgtacagaaaaatcgcatcagaactgtagagatgcgctccactactgaaacagcatagtaggcactgcttgacctaacacagtaatgcaagagtaaccaccaagatcaggaccttctaccactttcagagttgttttctgcccctacaactgttccctaacaccattacaagttctcaagtaagaaaaagaagggcagaggctccactgagtatctcctacaggcctgatagtggtattacctaggacatttactctgctcacaagatgggtagtggaagacataattactggacagcacaaagtctggaagcaagcagcagggcactaaaacagtgagagcttacacaacaaaagcttgttaaattaagtagtactgatgtggtgcaaatgaaatttttacagcaaaggttgaggaaggagatatgttagtgagaatcacatgaagcagactatcacaaaataaggccaccttcaaaatgttatgaactgtagaaccattctgatcttcaagtttggatttgtatagaggtttctgtataaagcattaatacctaatcaggagtttcctttagtgtgaacctttttgcatttgatgctattctctttgccaggaatgcttatctcccctggctcctcacttggcttgcttctttaatgtcaggtgttagctcatgcatcctttccttagaggctttccttgatgtcctacctgaagcatcccatctgttattctccagtacagtaccctgtttatctccttcatagacaagtaagataattaagggttagtgtaactgctgtctcagcaaaggcaggaactgtagttgtcttgttcacctttacccaaagactaagaaaagttcctggtacaaacaggtgaacaataaatatttgttgaatgaataaaaaattactataccaaatttacatgaacacatacatatacacacaaatataggaaaatggggagtacccaatagaaaaccaccaaatgttgaaagtattgaaaatgatacctatagagacaggtggatatgatttcaaagaacaagtaccaaagacagcttcaaaaatatgaaaatttatgaaaagacgaccaggagtggttattttccatttctactaagatgcaaacaagaagaaatgtttaaactgcaatgagtcaacatcagacataataattatttgctgcagaatgaactagcaacagagtttcggaaatctcctctcactacagagcatgaaatattgtcaatcacaaaaccaggatcagttaagaacagctcagactgcaggtaacttataagctaaaaaacttgctaaataaatggcttttcccccaatttttaaaattctgaattcataattatgtgtagaataacaatcaatttataaactgaatacaacatactttaaaaacagatggcccatatctgctgatcctacctcagcatcacttttctaggtattttgcagaaacaattacatttacaaaaggcccatttcataatgcaatctggttactaaaccaaatcaaactactcgaagagcagaaggtctgctgttgaaatattgtaaaatacctttggaaaaacggtatttatagattagcttttttaaaaagggataaatatgtggaagtaattctagcatatccctgaaaataattatactgccacctatgcattttttatgaggtggaaggataaatcaacagactgctagattatacaagccaattattcctgttgaaatttgggcataagacaaagggactttctccatatgaattcttactgtatcccagaattaactggtgccagcagtatcaatgcaactattactggtgatgatgtcatgttatgctgttttgattatgaggacaaaaatgggaatggaaaaaagaggcttggaaaggttttcagtatggtttccttataataagatttagcagttaaaaaaaaaaacaaaaaaaaacaaaaaaccacaaaaagaatgactgtttaagccccactgaacacattaaggtcaaggatttcaaaagttaatccacttttcttcccccaagagtttatttttggtaaaaggcagaaaaattagtttttctacaggaaaatctgcttctaaataatttgaaaatcttgatatatattatatattaaaaaagacacacaaaaataacagagaagtgggaataacagattaggtactgcaactttataaaggtttgcctagatcaagaagcagcgcacacacacacctcatctatgcaaactaaaaatgtatataaacagcacaatactgtgatactggatcatgatacattacctgtacacataactactactgttattaataaacctttgggacactcagttttatgcccaataagacatcattaagtctttaaaatcttctcttcctctttaatgggagagtatttctagacactaattttcccatctaatattcaaatataggaaacagattccacaaggtgctttaattgatgagacctcaagtgctgttttctctcttgaacttttggatagtaaacagtccatagggaccacacacaatgctatgacagaagagttgttacattaagtcttttcatgggacttgattggtgaagctttatgacatgcttgagcaacgcactgaaggggatcccatctgagttaatactttgtccaaccactgtagaggtccattcagatgaagttcaatccagcaaggagtacttgttaccgtctgccttcggtattctgctccccaccctttcacaaaactcattcttatggtgcacattctagttagctgatagacggcttcaaaaccctgattaacagactgagccagaagagcagcaaattcctggttgttgaagatcttcagattacagcctggtggaattttacacactgttgcagggtgccagccatatctctgattacaattggggctctgcacaaagattgcactatcacttaggcactcagcaaaaacttccccacctatgtagtataagcgcactcctcttcctatatgccttcttgtcatttctaccgtggcatttcggttaacattggagagtaaacctaagcagaacctctctgaatttgatgggtctgtaaagccatctacagtgagtgagggctgtgatgcatggaaggtttctccaaccctctgatttaattcataatatgctatcgaacaccaaaatgcaggttctgagtaagtaactggctgtaaatccaagctatgattaacaggggaaagagtagtaggagatagttctgctggagagcctgtgtccatactttgattcaactgttggtcacttgtttctccatcttcactgatatatccaggaggtggcgtttctggaatataattactctgtggctcaattcctgctgggaagttagtgttttctggaatggagtgagtatagtcatccagaggcggaagttctgttaggatctcggtgtgtcggggcactaatactggaggcaaaactggtgtctcaactctctgatagtggtaagggtttacacatacttcatcctttttaagattaaaagcatattcgcagttttcaattgccttgagttcatgatgactgtgaagatcaggccagcgccataatcggcaatatataacatgtggcaatccttttcgatgggatacctggagacgaccatcaagagacctggtttgttcagagaagctgtaaaggcctgttgtatcccactgatctatcgtatttggtgtactcagtccccaaatttcagagcaagtgcttggtatggtaacacatttagtattacagttttgagtggtgatggctttctcaagctcatctaatcgtcctgttttctttagcttcttcaccagacttttcactgctttctcacaccacttttcttcctgcccattctgctctcctccgcctgctcctccagacccaccagctgacttcttccatcccagcagtctcttcacaactggcggcgtgaatggcaagatggacgacatgttcttaccaaaggcagcaagccacgctaggaaaacagcctcttgtatcgaacctcccggcggctggcgggctgctggctggcgagctgcttctccgccgccgcggccgcgcgggtagacccgcct

SEQ ID NO: 11474 - RNA, 30222 nt, Homo sapiens
  source 1..30222: mol_type = other RNA
ctgaatagctgggactacaggtgcctgccaccatgcccagctaattttttttttttttttttttgagatggagtcttgcaatgtcacccaggctggagtgcagtggcgcaatctcggctcactgcaacctctgcctcccgggttcatgcgattctcctgcctcagcctcccgagtagctgggattacaggcacacaccaccacacccggctaattttctgcatttttagtacagatggggtttcactatgttggccagactggtctcaaactcgtgacctcatgatccacctgcctcggcctcccaaagtgctgggattacaggcatgagccactgtacccggccccacaatttttttttttttttttttttggagagatgggatcttgctatgttgatcaggctggaaacctgggtcttgaataatggatacatttggaagtgcagagcaaaggccagagagatatccaagccagagagatatccaaggcagaacaaagctcataatttaacaagaaaggtaggcatagataggcctaattatgatgaatgctctcttaccagtataaacaaattacaaagggagtgatgagaagaggcaatgaagtttggggagggaaagaaaagtctgtggtggaggtgataacctgaacttggctttgaggaataaagagttttatatcagggcatcaagagaaggatattcaaggtacttaggaccagaacaggcaaaggcactgaagcaagagagtctggggcaagaatgtctctattgggtcaagactttgacaatattaaagattccattttcttcatatatgcccccctgctgtctttccaataaaggtaagccctgaagcctgacagtcacaggaaaggagagggtgtgtactagagtaacagcacagttgctactcagctgtgaatctcagagcctgcctttattatcttgattattctttggcatctctaggaagatgataagtagtcttcaaagtcagactttactgagaatgagaagggagttctacatgctaagagctccattcacatactaaaagcaaagcttggacaactgaacatgagttttactcctaaccatggataagagaaactgagaatacgatgtgagaagagtctcttcattaggcaggagtggaatgactcccagggcagggagagattgattgagattgcaattgccctgttgggaaataaacggaaacttcaggatgggtatgcgagtcttggagcagcagggttagtcaactactttcctggcatagcctggggaagactgcaagccactcaaaaaagtcctactcatgacttagaggcttacccagtatggcacaggagcactagctcagcattggtggaaggaggtgtctagtcagtctgagaaaatgttggcttcccaaagcttgagcaagatgttcagtacatcccaaagttccaacatcatcccttcccacccactccaaagcccagcagattaacagtcccatagttgggacatggaagctattaaggtagagaccttgagaccaaaggcaatgacagagttgtggtcaggagcagggcatgacagcagtgaacaaaagccagggacccacttacattacccagtagactcagtgacatccagcaaagatggcaggatgagcaccagcagcaggaccgtcaaggacctcagcacatacattagagaaactctttcctgtgtcacctggagatgactgttctcacccactagatgccatcatgaggaagaagctaggaagaacctttgaaaagctgagcatttatccaaagagatggttttaagcctgagataggctatttgaatcgaaagagaacgttatctttgattggcaagtttaaggccatccacctcgtcccacaccttcccaaaaccagatgggatgcatgagaaattgatgtgaaatgaaggaactgtaacttcttttctgcatgatctgagttttaatgtgtgggagctgggaagagggaagaacattgatagaaaatctgaaagcccacagggaatgtggtctaaagcagaggtttaagtcctggctgataatcattttgggttttctgaaaatgcagatcccagtgctccaattccagacctgctaaagcagaatctcacaattgaggccagggaacctacattttagaagctctccttctgactccaatttggaaaccatttatttaaccactagtacaaaaactggccttgaataagacatcacttcctccaagtctgagtacagcacgcaagggcaactgcagcaaatggaggggtgatttagtaaggagggggtgaaaccgaaaatcaacaaggtttgtgtgaactggtctcgacacacttggctgtgaatagcagggatagaaagtagttatggggcttgcaaggacattgtcttaattttcctgttgtcttaacagaggatttactgagcccatgtatgctgtaggaaaaagctagtggtgccagagtttaagttttcagaggaggaataattgacctatgtatgagttctagagaagccttgcagacttacccagggctcagagcacatggcttagtcctgacataaaataccatttttcctctaccacttggctaagaagctgaggaggaactggcagtgagggaggaggttgagaatgaaagttctggagagtcacctaagagacggtaaacacatacctcatgtcttggcttctagagcccggagataagatcagcttcccttgaaaatgttagctcccatgccacatttagtcaagacaacaataacaaaaggctttcttcagggagggcagtggaagtgagtttgagataaaaaggaatttatttatttgcacctatgtattgttcagaagttttaggtcttatgaaaaaaagatttttataaattatacacaattgggtagctttaaaaaataccaaaatatacagtggtcaccctaaaactaacatttttggataatacacttataaattggaaaatgagaaaagatagtctggtataactgcctgaacaacttattaagaacattaacaagtaataacacatattttaatgtaatattgctgactaatttggcacatttaatacacgtccaatatattttctatgtactgtgaaagcttttgggaaaataaagcagcttgtgttacaaaaactgcaacctttcacaaaggttacccacaaaatacttttgcctagccactgcctgtccaacttcagagtggcaccacccttgctattgatctttgtaaccaacgacaattatttcaaaacaattatacaaccctcatttttctttaaaatctttgtcttcctttacttccctgaatacacacgtagtttaccatgacatgggtcttttttttttttttttggagacgtagttttgcactgtcgcccaggctggagtgcagtggcacatctaggctcactgcaacctccacttctcaggttcaagccaatcttctgcctcagcctcccaagtagcgggatcataggcacccaccaatacacccatctaattttttgtatttttagtagagagggggtttcactatgttggccaggctggtctcaaactcctgacctcgtgatcggcccacctcagcctcccaaagtgctgggattacaggcataagccaccgcgcacggcccatgacatgcgtatttctacagcaatgctgtattcccaaatagagttttcttttagagagcctctctctgtgttgacataaatggtgttcagcagtagaacctgaagtaggacacatttcagagagaagtggtgatctcagaatcagtatgcagtactcacaggagccctttgggctctccgcttacatagcttgtctgttctgccccagtgagtcttttctcaggcagagcctcccacttttggcagaggctttttgacttgactttggatttgtcttggttctaagaccactttaataaaggactttacatccctcctgggatgacaaaagactttttgtctttcctggcaagtcctttttgatataaagacaagtgtccctctggtttgagtactctggatttaaaaacaatttttttttagagacagtgtctcactatactgctgaggctggtcttgaactcatgggctcaagcgatcctcctgccttggcctcccaaagtgctgggattacaggcatgggccactgcgcctggctgagtactctggattctgaggcatgccttttctggtaaatttactttgggttcttctgtgtttatattattttttaatctgcatgactgggttaacacttttgggaacactgattttggtttcgtttcgatatggttacatgcatctgtaaatgatttggctcttttcccctgtttctgaacatctcccaagagcaaaaataaacattctaaattttgggcacaggatggctcttttaaagccactagggcaatcgccaccagttaaaacactggtccaaacacctgacttatctgtcaggatttacagaattttctttgctcttaagagattgagaagaaacaaaatggaaattctcaaacattaaggcatgcctgcttttctgggacttcaggtcagctatgtggcttttcctcatgcatgtttttggatcaatgaccatcatagagattgtctatgctttgtctaaactccccaagcttttttattcttagtaccaagagactgcagctatagagttgatatgtagagtcttctaagctctctaattttttttctgcctactttaaatctgctgtttctgccagtgttgagatgaaactcactccttacggcattccagccaagaacaaaaagaaaaaaaaaggtcttaaagggccttaaattaatggctttataaattataatagttccctggcaaccaacacctagaattaagaagtatcccttttaatgtaaatttaggtttgcctaataactgcttagggtgatggaacagttaattaaaggattaatagcctaaaagaactagataaatacgtataaaaattaggctctcaaacaggtcaaaatcttgagctcagggcaataatataaggtatctctggtatagcataaaaattgcttgcctgctatgcaaaggctaaaagaacaaaacaaaaacccctcatccacaactgctaaaatgcttccctgcctgcactgactagtcaaaaaaaccagaatggcaaacaaaagatttgttactaaaaattcaaggccacctggagattgttttttcttatacaattcagccagtcctagctaaaaatgtaagcatttaaatattaacattaaactcatttgaaactgaaaaaagggaaaaaaggggttggggaggtggggtaagaggttttttaaaaatccaaactgctatttaccaaaacttttggttcacagctttcataagattacctattctgcatgtttacccagctgagcaggtcccactttctcagaaatataatttgaatccaataactgtcttttataaaccagcaagcctgtattactatcgtatgactaaaattctaaaatgaaagctatgtttgtgtatgtgtatgtttaggtgtgtttacacatatgtatatatatgttgtatgttgtgtctacgtggtaaaatctggcagttggccacaaatcccttaaggaattctattcatcaaataaatgagtgctaatacaaaatatatagtaattaacacaagtgccttttagttaatataacttaaacatctgataagctggttttaaaataattggtaaatcaaaaataagtgtctttaaaatttttgcctgaatttactactcagttttatatttgtctctgttagactttttaaggtcataaaactataaactcaacttaaaaacagaatgatctttgtataactgtaagttgaactaattttgtattattgacttcagctgtgtcctctgagttactggcaaaatacctacatatttcatttttatggttcttaattgaacacatgatactcacaggtaataaaaatggttaacaggaaaataacttgaaatgactagctatgtctaatatctcagtttttataagtaatctaggaataattgttaaaaatgaattgggggccaggtgcagtggctcacgcctgtaatcctagcactttgggaggccaaggcgggcagatcacgaggtcaggagatcgagatcacggtgaaacctcgtctctactaaaaatacaaaaaattggctgggcgcggtggcgggcgcctgtagtcccagctactcgggaggctgaggcaggagaatggcatgaacccagaaggcggagcttgcagtgagccgagatcacgccactgcactccagcctgggtgacagagcgagactccgtctcaaaaaaaaaaaaaaaaaaaagaattggatggattataaacgggataagcaagggtgagacatggtggtatgcaggtatgcatctatagttccagctactcaggaaacggaggcaggaggattgtgtgagttggagtttgaggctgcagtgtgctacaattgtgcctgtgaacagccactgaactccagcctgggtaacacagcaagacattgtctctaaaaaataaaccaaaagaatgtttttaaaaataggatgttaatgaacttttcatgtaatttgaaatcttataaattaatcttcagtaaatgtctggatcatttccaaaaaaaaacaataaactgctgaaaatattagtttgttcttggcttcctaaattatagaaagactaaatatatttgggcctattaatatacaaagttataaggaaacatgtttctaaaaattataatatggttctcatttataaaatgctgatataacacttcaaaattttgcttcctaggttttcactaaaaattaaggttaataagttaaaatttgaaaatacacaattccatatacaaagtgtacccaaaaaaagatgttttgatgagaaaagttataaggcataaaaattgctttttattgggaaaaaagttgtttaaattcagagtttattagaggttgtttcaaatatggaaacaagacagaaaggaaccactaagtaggaggaggagagaaatatgaaggaagttaatgggtgtgagaatgtacctttggtaaggaaggttacaaaattaacagaataattctgtatgagtcttgcatagtaactttttatcctaaagcaggatgaccagttgtttaaggggaagtataaaacaaagcagaaagtttaagcatgtcactgaaggtctgtgcagatcatgaaatgttcatgaaggatacatttatgaaaggagttgtgtgtaatgaagttggcaataggtcagaatgaaatcataagacattgagcttacatatatacttgtacatatgtatatgtacaataatacagtatattctatacatatgctatatatttgtatatacacgatagtgtaaatgctatacatgcactatacacacacacacacacacacacacacacacacacacacacacacaaaatttggtccccaatgttagaacaaggttctttttaaggatctggtcttaataaaattgaaagaggttttaatttttaattctaaaatcagccatcttctaaaccacagtttaaatttctgccatatttccttctgagatccgtttaatttcccctagattcaggttagaaaggctgtcttttttcatttaagatggtcatttcatttcttgaggtagagttttcttcttgaagatcctgatttatatctcacaagttcaacctttgctgtatcttgctgcaccttatttgtaggtcacacatcattgcctttagctctttctccccttaagaaggtacatctttttgtttggcaggggtgataactcttaactttttcattagctcctgtaacttttttcctctggttctaactcttgctgttataacttgatactgaaatgttctgtagaaggcctagaaaagcaatgttttcctccagtataacttgattctgaattcttggctcttctcatgtttgaattgttccacgcaagcaggaaatttctcgtaatttttccaagagccatgtattctgttcaacatactagctttcttatttacattcctctataaggcgtacactcataaccttggaaatactcttcctgtgtctgattaaattcaagtaccttttcatcagattcaactttcagtatatccaaataggcttcccataagtaaaggcagtcacactgcaagagatttttctttaccattttggcaactggcctaagaaaaattttatgttctatcaagataaattcttgtgtttaagttttttttttgcttgggaaaaatgaagctttgaaaagatggtttttaaatgtatgtaactttctgcattgcttcttaagtcttttgattatcattcttgttaaatattttatagtgacctgtgatcctgtttcgaacttttgacatctttgacaggcttctctaggctcaagttctaaattaagtgtttttgacttaaaattacctttgagttttccacttgggcctctggaaagcctcagagcatgtgtatgccatctggtagagatgttagctaattaggcttctttgatgtattaaattgtatgaaaagcattgtctaatgatgtaatactagacacagttacatttatgagtatgttattgatatgagtgttccaaaattgtacgatgccgttagaaatatgtcatcagtcataattctgattatgctgtttgccacaaaaataaccaaaactctttgtctatttctggttatggtaaactctcatcagatttttaatcatggttattctaagtttttgtaattcccagttattgctttttctctaaaagcatttgcaatcagattcatggaaaagatgctaacacacttttaaatacaggttactaatcactttaataccaatggactaaatattttttcagaacttcaagaaactgatgagtccatgtaactactaattaagatcaaccacaacaaaaaaagttacatgagactaagtaactgaagatgtgtctgtgacttttatttgaagcattattgtttttttacttaaatgttttgttttccatatttaaagaaattctctcatgctatctatagtttacagcaatttggaatacttttgtgaacaaaggtagaaatatttgcttttcctttcttcttgatccctccaatttggaaactattttgagtattcatttgtttttgtttttgagacggagtctcgctctgttgccccagctggaatgcagtggcacgatcttgtttcagtgcaacttctgcctccagggttcaagcaattctgtctcagcctcccaagtagctgggactacaggcatgcaccaccacacccagctaatttttgtattttttagtagagacggtggccggggggaggtttcactatgttggccaggctggtttcaaactcctgacctcaggtgttccacctgtcttggcctcccaaagagctgggattacaggcatgagccactgtgcccagcctatttgtgagtactcttaaggcaatatgatttgcctaagttcaataaaaatcggctctcgttataacaggatacaattggaaacactggttgtattaccaaggctttgattaaaatgtcatatttgagaatgtgtagaatgcctggcttcaatggttctcagcattacactgaattaaaaattatcatttcctggcaggcccaggaaccttaaaactataggtaaaatctaaagtctaccttgacttagcttcttagcctcaaggaggtttttaaatctgagattactgtgaccatactactattcttgcagacaaaatctgataaagtttacaaatctgttttattctgaacatctttggtaaaaatcagggtaactttaagtttctgaagaaagctatatgtacctgttattagatcacagctctgtaccgttttgaaactcctgttatccacctgcagactggatttgctcctgaatcctcctaatttccttcaatatttggctatgactctctaagaaaaaaaactactcccatgctctgaggcctataagctaagatgtgattaatttttaaaggagcaagtctcatgctgatgtatgggtcacacaaaagttcaccataccaaccaatgccatagctagagacattcaaactgcaaaccaggacaaaaagttgatgatttcaggctgtagacatttttcctaagacatcagagcaagaattgtattacaatttgatttattcaattggttgcctgtaagcctaggttcagggctcaaaaccattatgcaaactgggattgtcacattactattaattttgtgtatttcctttttaaactttgtatctgttatttgccaaattttctgcagaaagaagtacaattcctaacagaataatgctagcccagcactttgaggggacaacaaaggactaaggaaaaaaaattggacttaataatagactccaggtggacttagcctaagtgccactcccttaaagcctccctgccctcaaaggtggctaaaagggttttaacactgacttttagttgccaatcactcctgccaatgcaggatgcaggaccagaccaataacccgggaaaggtctattctgtcaccaagggacaatcaaagcctaactacaagatgattcatcatagatactttcggaaaaacatcttcatcaagagagggaaaggtgaaagctgtcagaatcaagagtcatgtttccaaaagccctgacaaatggagccagggaagtccatgaagagagggattttacgcactacctcaaagacccagaagaaaccacgccagcttgcacaaacactattcgcaaccttacacagaaaatacttttgggacatctgcctagaagccgattgtccaaacccgaactggcagcatccttgttattaatccttgtagccaagaataattatttcaagacaattatataatctttatctgtcctttaaaaacctgtcttcctttaccttcctgaatacacacagtttactatggcatgcatattgccttcacaatgccctattcccaaataaacatcattttcttttagaaagcctctgttatttaggttgacagttattacacctgaaaactaaattctagctgatcaataaaattctttggttctactgtatacttttatttggggatatctgcttccaaacacactaaagtacagtatactcaattttaaatatagacagtatatttaaaaaaaacataaaaagtatgtcgaacatttttaatttcaaacaccaaacttaaatagactaataacacagatcttctgtggtccacaaatcatggcaaaaaactttgttttcatatgcccattatggcttgctgactggcttactgcattttagattttccttatgattttagtagctttctctaatggaatgtgctgtgagtgaagcttcaaacattttccattgaatatacacagacatacaaataaagactggaaaaaatatacaccagtcgttttctctggttgttggaatctgggtgattttttaaagtcccatccactgggctgccagtaaaagaccacaaaatatttttgtgtatttacaggaacgtgataatcaaaagttgttgtgggaccattcaagatgagcgtggggaagggaagcccatttaaacatatattcaaggaaaaatatattaagttacctgaacatttgggtagaaatactgagcactgctatggtctgtctcccaaactgtccctcaaatgtatgatgagattttatcttcattgtggtggtgttgagagctggggcctagtgggagatgtttggttcactgaggcagatgcttcatgaatggcttggtgctgctcttgcaatgagttctcactctctcaagactagattagtccccaggagtgggttgttaaaaagagacttgtttggttgttgtgaacaagtgggttgtttgcacgtctgcttcccctctgaccttctccatcaagctatgaagcagcagcaaagcccttgccaaaagccagggccatgcccttgaacttcccagcctgtagaactgtgagcatccttcataagtgaccctgcctcagctatcctgttatagtaacacaaaacagactaagacaggcacacaaaagctgaggactgctgtcgactccactttcaagggctaccaagcacagccacatcaccaaagagaacaattcctgacctccttggaagcagaaacttgactctccgggcaagataactgttgtctttttaaaatttcagtgtcaaagttaaaacatgccttgatcagtcaaccaaattactgctaaaccagtattgggaagcttcctaaagcactccaagctcctaaaaacaggcagcatgaagtaaagcagatagcatctttgcatttaagaagtcccagaaaggttttggaaatggcattaatgtaaatgttcacattaagagaaaacggtttccctgaattgagtgattctttctactttctagtgctgtacaggataggctcagcgtttggagagtgttaacttccagtcatgtgataatggccaggagcaaccacaatgattaacctttagatagaaaacacaatcctttgcttttgtcttccttatgtatattagattaggcttctactcaatgctctgtaagttaaaacatttcaaaccaaataggccactctattaagtcccagcttgagcattcttcagcttctccacattttccattgtttgctggcaaaccagtacagtaacctgttaaatacaaagcaagggtgtggtagattgactgcatttaaggctccaattcttcacccctcctatgttctctcccttggtctaataactctgtagtgcctttccacactgggtttagccatgtggcttgtttctggtgaatgctagttagcatgaagcatgcagacatgaaagggagttatgggattgggcttggctgttgttgccttctacaacctccacaaaaacatgcttgtttaatggaggataggaggcatgtggaaaaatgccaagtccttccaggtgaggccaactccctcatgaacgaggaaagactacaactgctccagagacatctagccgaaatcacttatctaattcataaactgtttattgctgcacaccactgggtttttgtggttgctacgagttacttttgcggcaataattgctccaatatgttctatgtgacatttctgagtttaacatcacatttacaaactttcttagagaaagatttgttattagcaaagaccttcagagtaacctttgcctggtattctagactgtgcagatttagccatctaatactgagtacccacttcaggctgaatgatctctcaagtgctctcatttagttctcataaccaccctaaaaactaacttcctcattttagggaactggaggaaatgaagaactttaaggtagactgatgaaaagatttatctaaagtcacataaattggcacaatcagggtccaaaccccaggcctccgattctgagtcaaactgcattttccattacatcggaaatgaccaaggattaaaattagcagaatgttattctgtccagccattaaaatccaaaaaaaaaatttgttcaaagtaggcaattgagttttcattctattatccaaggtaactgaagtatttgactgtacaggactgcttccttcaagtgttccatccttagcattcttgttaaaaatggcctttaagatattgctattcccagtcaagaaatacccagacaactaaagagactaaaatcatgtaaatcatccatttcccagttgaatcttaaaaaaaaatttatgctcaatacctctctccagccaatcactatgtaaattgtgaattaagacattattacttggtggcaataacggttagaaaaaaagcacatccctctccctctcccgtctccccccgtctcccactttctacggtctcccactttccaccgtctccctctgatgccgagccaaggctggactgtactgccgccatctcggctcactgcaacctccctgcctgattctcctgcctcagcctgccgagtgcctgggattgcagacgcgcgccgccacgcctgactggtttttgtattttttggtggagacggggtttcgccgtgttggccaggctggtctccagctcctgaccgcgcatgatctgcccgcctgggcctcccgaggtgctgggattgcagatggagtctcgctcactcagtgctcaatgttgcccaggctggagtgcagtggcacgatctcggctcgctacaacctccacctcccagccgcctgccttggcctcccaaagtgcggagattgcagcctctgcccggccgccaccccgtctgggaagtgaggagcatctctgcctggctgcccatcgtctgggatgtgaggagcccctcagcccggccgcccagtctgggaagtgaggagcgcctcttcccggccgcccatcgtctgagatgtggggagcgcctctgccccgccgccccgtctgggatgtgaggagtgtctctgcccgaccgccaccccgtctgggaggtgaggagcgtctctgcccggccgccccgtctgagaagtgaggagcccctccgcccagcaaccaccccgtccgggaagtaaggagcgtctccgcccagcagccgccccgtctgggagggaggtggggggcagcccctgctcggccagccgccccgtccgggaggtggggggcaacccccgcccggccagctgccccgttcgggaggtggggggcagcccccggccagcatccaccccgtccgggaggtgggggggcgcctctgcccagccgccccgtctgggaagtgaggagcccctctgcccggccgccaccctgtctgggaggtgtacccaacagctcattgagagcgggccatgatgacgatggcggttttgtcgaatagaaaagggggaaatgtggggaaaggaaagagagatcagattgttgctgtgtctgtgtagaaagaagtagacataggagactccattttgttctgtactaggaaaaattcttctgccttgggatgctgttaatctataaccttacccccaaccccgtgctctctgaaacatgtgctgtgtccactcagggttaaatggattaagggcggtgcaagatgtgctttgttaaacagatgcttgaaggcagcatgctcgttaagagtcatcaccactccttaatctcaagtacccagggacacaaacactgcagaaggccgcagggtcctctgcctaggaaaaccagagacccttgttcacatgtttatctgctgaccttccctccactattgtcctatgaccctgccacatccccctctccgagaaacacccaagaatgatcaataaatactaaaaaaaaaaaaaaaaaaaaaaaaaaagactttagttcaagttgagaccaaagactgtgctattatggggtggagaaaagtatcacaattttggtaatactaggcaagatgtaacctcaagtctccaggcagccccatgagcttccctgtgaatgagaacagaaaaagttcaggagccaccagaggatgttaaggaggcttcctagagaagacgtggcaatgcacctgatggagacgtttaatttcttcactacaaggaatttcaaacttatctaaaaggaaatagaatacaacaaagctcccttacccaatcccaacaaacaaccatcaatgtcctattcattcatacctccatctacttcctctgtcacatactattttgaagcaagtcttacccattgtattttacccataaatgtttcattctgtatctctaaaacattgtctctagacctcagcaaaaaaaaaaaagcacatccacttttacaatggtcacatacaaatggggaaagagtggatataaaaaatatgcacccaccttcaatcaaatgcgatcttttaaagaatataaacaagccagattcttaggtatctctcccttttgtaattttgattctgaaaaaatatttaaagtaatcaattaggtattctaaaagaaggcagttttctaggggtttatttaattataggggggttggggtagagagattaaaaacgggaagcagtgcataggcagtatgaagtagacactttggcaaataaaaactgcaccgtatgacatgtcacatagaaattgttagagactttgaatcctaaaatttagtttaccaaatgtagctttttatgttttatgttttaccaacaaataatttgtatgttaaatttaagcatctgaattccgaaatgataaagaacaggaaaataatgactaagctaacaaccaaactttcagagtataaaattttgtcagtggttttcattttagaattaaaaatttgaatttccctttgcctacaagtctaagtaacttgcagcagcaaattcccccactgacaacttcaaagcatagcaagaatccacagtggtttgcaggccactaattcttttacagatgaaagcattcaattatctctataaaattcaattccttagaatatgtgtttgtgattgacgatgtacatttttaaatgtggtgataacacgttattattcatgatttaaaagttgaaatgaagtagcttgtggttcttgggtaaaacagacactaataagttttttttcaatataaaagagcaacctagacattcctataaaacatttttattccaggtggtaagctggcttaaattttcacttttcagccaggcatgatggctcacgcctgtaattccagcactttgggaggccgaggcaggcaaatcatctgaggtcaggagttcaagaccagcctggcaaacatggtgaaaccctgtctccactaaaaatacaaaaagtagttgggcgtggtggtgtgtgcctgtaatcccagctactcaggaggctaaggcaggagaatcacttgaacccaggaggcgaggctgcagtgagccgagatcgccccactgcaccccagcctgggcaacagagcaagactctgtctccaaaaaaaaaaaaaaaaaattcgtttttctcacagcagcacatttctaaatggcaaaccatttagaagtgagtcatcatttgtattaaaatcttatttacatggtacttatgtagtttgatcaaatactgccacaatatagtttagaggcaagacctctcatgaagaaaaactttacaagatttaaaatcagagcaaatgaatttcttaagttcaagatacgtactctcaatggagaatcgctgttgggcagtggttaaggcctctgatttgctacttattagaaaaatccacatatatacaaaactctgctaaaattccaatggcttctctagatgaatcatctttggctgtgagcaaaaaagttaactaagtttcacttaatacacacacacacactagggtttatatgtagcaacttcctcatcctcattccacaggtagcccgttcttggctgggttatggcttgtaatctcagaaccactgcccccaaatgactgctcagaagcacaatctcactgcaaactatggaacccaaactatacagctatccttggcttttaactccaagctatctaggccttgtgattatatgtgggcttcatagcagaacctaccaggcttgtggttatcaattttctgctcaccatataagcagtagctcaataacaccgtccagttttcatgtatatccagacacacaggtgagagttctgttccaagatctcattttgaccttcttcaaaggtcttctccatctctccaaattgaatgtattcttcaaccctgggcttactgtattctgcccatcttcttcctggaccaaactgttcagaagttaacttctttttcctgtcatcacatctctttcctaaactactttagaacttaaataattttattttcacataacatttagaaaggtgcagaggcagccaacaaaactattgaagacagactgtaaaaactggcaaatccccatctcaaattccatttattctataaccaataaagtcatgcagtttggacgggagcacagtaatacattctgttctcatgtagcttcctaagtatgcttagtctattgttcatttatcactgaatctgttatctgctaagtctgattcaatgttcttgccttctattaatgtgattttaagaattactgcatgtctcactatggcaaaatagcatgacatttgttttacaaaatcagttaaaccaattctacaaatatttccatacctatttattgcagcaaaagataatttttatgtgtaaattagctttttgggtttttctattcctttatttgtaaacttataatttttaggttgggcttactattttgatgagaagggtgaatctgtcaaagggtaagctggataactgtatgttgcaaacatgttcctgaacattcttcacccaaacttagacaaacctggagcttaaaataattacattggatgacatcagtttgatactgatgcctgcttcctgcactaagaggctttcaatctattttgaagagggaaaaacagaatatgccaagtggggagacagcccaaacatagaccttaatacttctctcatactcttcagccatttgatgaacatgtggaattatggatgctagggccattataaaaatctcctgatacagaacagtgtcactacttcaagctaagcagtgacaggcaaagccaggctgaggtgacaatgtagaaggatctcgagtcagccctcaatgttgttgttcaatgttgggaagtcccttttagattatttatacagtggcaggtggtagcaattacagtaaattttcttgggtttcttcctaataaaaaagtgttgataaaactacaccagtcccaaggctattcaatgccacgtaaaatagtgtattttagcatttgaggtccctttttgttgcatactaaagcatgtttaaaatggtttgcagaaaacagtctgctaaccagtactgattcatccacagaactgaattcttgcaaggcacaaaggaagtgtggctgacctaaatatttctcatttttaaaattattcatactgattatatgagattatatcttatctagtatttttcaatggagccttaaaaatgttattttgttaaaagtatatttcagcaaatttcaactttgaagatgtttttgtttacagcatagatcttatgtattagagcgctaatgtagcataggcaaactctgaaataaataaaaatgtataaatagcactgtgcagtgtgtggtgtgcgcctgttgtggggttatattaagtagtataaatttatctcccggggggataggataatcttttatgtaacaccaaattaaaaaaacaaaaacatgtactcttaaaatcatatgtccatatgtgaaatacaatcactttttttggtttccatataatttagggagtgaacaccaaaatgtaatcccatataaaaaaagatcagtttaaataaaaattaaaacaattaaaaattagtcccatagtaacatggtaaacaactcaaatggctttcttttaatgctaggaaaactgtccacctttcaacggtgacagggctgttaacacaggtaagagcaaacaaggtaaaaagtgaaagcacatacagatgatgcacacaaatatatataaaaattgaccagaaatcacaggacatgtaagcaatgttttcttaagcagaactttttttgtactttaaatagactaaaatatttggtgtaggtgggagaaagacatcagtattcaacaattttaacttgaaaaccagctgtaataaagcctcagctcattgtttaataaaaataaaaaaggaaccacatcgtacttttgacaatcatagaacgaaagctcacaaagaacacatttaatatctccatcacagtgcaccaaggatgcagccactaaggacttccagagggaaacaagaacagggtctgcatccatcatattgcattacaaagttaatgccatcagagaaaaaaaatctcacctcacgtgctcaatgttctagctggtaagcaccttatgagtatgaggctacaattgagagaaactgctcagtctgcatcaggacacccaattccttcacttgccattggctgatgcatttaatcattttaacacaacattcacggaaaaatgttaacaacacattctggcttctcgagcagaacagactgggaaatgcagtagacgccagagcatcaaaggccatgtatttcctcacaagaaaagaaatctgcaacaattggtttccttttactatgaaaaatgtaaatttcagattaagtttaaccccataaggacgcatgatttgtacttacatatacacataggttcagaagaacttagctatctagttggcctcttctctgttccattataacatcagttaccttagctggatcactaagtgtgagtctcaccaccatactggtaccttcagctattacctgtgttataaatctcatgttccattcaaagtactaaatgactggatggcacatatcccaataagtatcagaaatgttgacagccatagtgcagctgagtttagaagcaactatgacaacatagggaagtaaggataaatcacaagaacacctaaggtggtcagctccttctggtgtgcctgggacttgttttgagtttagcaaaaactttacaagattaaaaatcagagcaaatgaatttcttaagttcaagatatgtactctcaatggagaatcgcttttgggcagtggttaaggcctctgatgtgctacttatcagaaaaatccacatatatacaaaactctgctaaaagttttgtatccagggaaagtcccgcatccagggaaaccctcaatcccaggcactttagggcagctggtcaccctgagaacactacccactcgttccttaatatcactagagaaaaggtaagaactttcaagggcataacctttaagggcatcagtccccaaaatatttttacatcactagctaatggctagttcctctaagcttgctaaaaggctaggaagtccagaaataccttaaacgtgttaactttaagaagagttggtagtaatcaagcaaattagtgagcagtgtataaaagctcactcttgaaatctgttttcagacaaatcttctaaaggttcttctagctttgtccagttatatggtattttactgtattctctttttgcaattaatccagttttgtatgtcttttctttcttttttaggtgaaaatattctatgccaactgttttccacagtcctgcattatatattaaaacaaaggctgccagctggagacacagccctccgattacaaaggcccagaatgttacttttaactgtgctccaccaggaggtctggccttgggaaaagatggcgaaaggaatattctcagatatgaacattttttattctgcctacaatgctgtgatctagttcaacaactgcagaactgttctcatcttaatcgctgtagtttttctttctttactcttttgtataaaaggttagtgtcacagcttcactatcactaataaaaagatacaaatatgcctttcaagtcagggttggaaaagcaaaactgaggtgtgaggttacactggtctaagaaagtaccaatttgggttctatattttgtcaaacagttgggtttttaaaaaaattcaaaactcatgcatgttacctacttgtcatgtgtgaattatttctcacaattttaattaatctgtgtgtatattagttatataaagcaatggatttccacattcttaaagcaggaacctatattcaccagaaaaggatcctcctgtttctcatcaaattttttttcagctcgaacaatccaagattgggaatagtaagagtggcaaacaaatgttttcttagggacttactgagaaaagaaaaaacttactgggagaacagagacttagtaaaatttctattgctacagacaaatgctaaaaaccagctttataataacagcattataaaggatagaacttaatatagaaccagaaatatggcaagttacctagtgattaacattgtaaaatagtcaaaaactttaaagccacagagaaaggaaaacaattatgaaatggaaaatatataatatttaagtacttttataattctaaaacttcacttttgtccttaaatcaatatattacggatttcattgttcaataaattaccatctttaattaaaaataagtaaatcaaagagcatatttggagaaactaagagctgttaactgtttggagggtaaaagaatacttttctcgaaatttttttgaagaaaaatctaaaagccctctatgttgagttaatacaccttctgacccccatcatcagtggcattattcttccaagggactcttatatctaagcaatggtgaagttctggattcattatggatctcatggcaccaaaccaactggcactgaagttaagttaatatactccagcgagatcacctgtgggtcaaggatggcccagagaatcttggaaaatccatttatattgagcaaagatctgaatcaccttcaatcaggctgtaagatactagaaaatttgaccttgtagtagtatttcccagggtaacttaagcagcaaccttgcaccagaagaagaattaaagagggagcaatctagtattatcaacaacaacaaagttaaccctaagttagtacatcccagaatctgctggatgtataataatttagtaacggggtatatggcagagctttctttgatgttaacaaattttggctgtgattcttagttaccaagttgccaaaaaatggtatattaaatgaactgccaaatggcagattaagaaaattaatgtactccaatggtctgtccatgaaaggaaaatgtacacagacaaattaagaacattttaccaggatctgagatttaaacaatggaacaattgttttaactgttagaatgaccccaactgttaagtttgtctatgagtgtatatgtatatataaattcatacacatatattatttatttccttcttaaaaagactgaggcagttctgctatatatagttagctacaatattcaagataaaacagttcctactcaaaaaattacatgaacacacgagataagttcttatcgtaaatgctatcatgaggctatctagtatagctcatatttcctggttgtaaggctcaaaacacaggaattccactccaagagataatttgcccctcaatccctacaaagtgtagtctaaacaaacaaaatggtaataaaaaattgaaaaggaagatataaaaagaactcaatagcaggattctgactacctctggagaccacacactatcattattctgactgtcttaaatacaacaatccaatatgccccaagatggaaatctggtatcgtagggaaaacattggctgcaactgtcagaaaagttcataatcttaaacataatttatgccatttgccagtcacaaagacatttactgaacagaatttttgagccatttgtaaaattaaaatgattgatcaatttgaatagcaaccttcatgatgaagaaattaggactctaggtatgaaaagcatgttccttttttgttaataagttcaaaggagagaaacattctgatatatgcagataaaaatatggctaggctgggcgcggtggctcatgcctgtaatcccagcactttgggaagccgaggtggacagatcacgaggtcaggagatcgagaccatcctggccaacacggtgaaaccccgtctctactaaaaatacaaaaaattagccgagtgtggtggtgggcgcctgtagtcccagctacttgggaggctgaggcagaagcatggcgtgaacccgggaggcggagcttgcagtgaaccaagatcgcaccactgcactccaggttgggcaacagagcgagactccctctcaaaaaaaaaaaaaaaaaacaaaaaacaaggctaacaagaaagaggataaccagcaagtaccacctggatgtgtgttgtcaggtagaaaggaagaataaaattcaggcaatgaatataatagatttagcaaagtaaagcatatgaaaggaagaaatgtttgatatgtctaagtatcaatgccttcgatcagagtaagaaaaaagtattcattgttcatgtccacagactagatatctaaagagatacttggtgggcaggggcttgggagggaaggcgcaaattggaatgttcagcttttaaagtaaagactgtacatgaagacatattttatgtacagtgaagattgtcttgtgttactttatatcccaacataaacctacgccaccctcagacgaagagggtatctaacactgaataaatgctgaacctatttagtagttaaagaaaaaagagaaggatcttaaaggtatatatgggaagcttttaagaggtagagaaaccaactgggtatatattttcttttatttgatttcaactagcaagagactaagactgatgtttgtttgtttgttttaccttcaaagtcttagtcttaaattgacaagggcacaaaaaaagtgaaattaaaataattttaacaaaagggaaagcatttgacagtgtttaaaagacagacaaatcaagcaaaactcaatgtggcttaaggtaaaaaatacaactaggtattaaacaatttgtaaaaacttacaaagaaaatttagctttcaagaaaaattaggcagatttccttctgccaaagtgacaggtcctgaggaaaaaaaacacaacctctacaagaccaagcacagctcaagggtcagggccccgtcctagtcatctttttattattcaatatccatcacagtggctgggcaaacaacaggcatcaataaatgtttactaactgaatgtgtattataaggtataatcggtataactgatatagctcaaatctaatcatgaaagcttctttaaagtaggataaaaagagcacaatcagcggtattccagaaggtaggcctaaatccagttatatttttctaatcgttgaccagtggttataaagactttctgagcttctttttaaagcaatgaaactctttccaaaagaaaccccatgcagttcttcagtacagaataaatatgccactaagtcagtgagaactccaacagcctcccctaagccagcccccaaggtgtctctgtggaacctactggaaaaaatattactcatcttagaaatgtgatagaaagcatggccattcggttctcaggtcatcattcctagaaaattaacagtattgtgaagaataaatcctaagtaatgttgctaatttaaataaagacaaaaattcaacaaagaggggattctatcacttagaaaaatgaaaaccacacctataaatggggggaggggcagaaaacaaaaaaaaaatcaggccacagtagataaaatacaaaaaacatcatctcgttaaaaagcatcaaacacattcacacaaatgtaattacaaccaggaagtaaactgctcaacaggtataactgctcaataggtgttttcaaagagttgagtcccaatttcatactgtacagaaaaatcgcatcagaactgtagagatgcgctccactactgaaacagcatagtaggcactgcttgacctaacacagtaatgcaagagtaaccaccaagatcaggaccttctaccactttcagagttgttttctgcccctacaactgttccctaacaccattacaagttctcaagtaagaaaaagaagggcagaggctccactgagtatctcctacaggcctgatagtggtattacctaggacatttactctgctcacaagatgggtagtggaagacataattactggacagcacaaagtctggaagcaagcagcagggcactaaaacagtgagagcttacacaacaaaagcttgttaaattaagtagtactgatgtggtgcaaatgaaatttttacagcaaaggttgaggaaggagatatgttagtgagaatcacatgaagcagactatcacaaaataaggccaccttcaaaatgttatgaactgtagaaccattctgatcttcaagtttggatttgtatagaggtttctgtataaagcattaatacctaatcaggagtttcctttagtgtgaacctttttgcatttgatgctattctctttgccaggaatgcttatctcccctggctcctcacttggcttgcttctttaatgtcaggtgttagctcatgcatcctttccttagaggctttccttgatgtcctacctgaagcatcccatctgttattctccagtacagtaccctgtttatctccttcatagacaagtaagataattaagggttagtgtaactgctgtctcagcaaaggcaggaactgtagttgtcttgttcacctttacccaaagactaagaaaagttcctggtacaaacaggtgaacaataaatatttgttgaatgaataaaaaattactataccaaatttacatgaacacatacatatacacacaaatataggaaaatggggagtacccaatagaaaaccaccaaatgttgaaagtattgaaaatgatacctatagagacaggtggatatgatttcaaagaacaagtaccaaagacagcttcaaaaatatgaaaatttatgaaaagacgaccaggagtggttattttccatttctactaagatgcaaacaagaagaaatgtttaaactgcaatgagtcaacatcagacataataattatttgctgcagaatgaactagcaacagagtttcggaaatctcctctcactacagagcatgaaatattgtcaatcacaaaaccaggatcagttaagaacagctcagactgcaggtaacttataagctaaaaaacttgctaaataaatggcttttcccccaatttttaaaattctgaattcataattatgtgtagaataacaatcaatttataaactgaatacaacatactttaaaaacagatggcccatatctgctgatcctacctcagcatcacttttctaggtattttgcagaaacaattacatttacaaaaggcccatttcataatgcaatctggttactaaaccaaatcaaactactcgaagagcagaaggtctgctgttgaaatattgtaaaatacctttggaaaaacggtatttatagattagcttttttaaaaagggataaatatgtggaagtaattctagcatatccctgaaaataattatactgccacctatgcattttttatgaggtggaaggataaatcaacagactgctagattatacaagccaattattcctgttgaaatttgggcataagacaaagggactttctccatatgaattcttactgtatcccagaattaactggtgccagcagtatcaatgcaactattactggtgatgatgtcatgttatgctgttttgattatgaggacaaaaatgggaatggaaaaaagaggcttggaaaggttttcagtatggtttccttataataagatttagcagttaaaaaaaaaaacaaaaaaaaacaaaaaaccacaaaaagaatgactgtttaagccccactgaacacattaaggtcaaggatttcaaaagttaatccacttttcttcccccaagagtttatttttggtaaaaggcagaaaaattagtttttctacaggaaaatctgcttctaaataatttgaaaatcttgatatatattatatattaaaaaagacacacaaaaataacagagaagtgggaataacagattaggtactgcaactttataaaggtttgcctagatcaagaagcagcgcacacacacacctcatctatgcaaactaaaaatgtatataaacagcacaatactgtgatactggatcatgatacattacctgtacacataactactactgttattaataaacctttgggacactcagttttatgcccaataagacatcattaagtctttaaaatcttctcttcctctttaatgggagagtatttctagacactaattttcccatctaatattcaaatataggaaacagattccacaaggtgctttaattgatgagacctcaagtgctgttttctctcttgaacttttggatagtaaacagtccatagggaccacacacaatgctatgacagaagagttgttacattaagtcttttcatgggacttgattggtgaagctttatgacatgcttgagcaacgcactgaaggggatcccatctgagttaatactttgtccaaccactgtagaggtccattcagatgaagttcaatccagcaaggagtacttgttaccgtctgccttcggtattctgctccccaccctttcacaaaactcattcttatggtgcacattctagttagctgatagacggcttcaaaaccctgattaacagactgagccagaagagcagcaaattcctggttgttgaagatcttcagattacagcctggtggaattttacacactgttgcagggtgccagccatatctctgattacaattggggctctgcacaaagattgcactatcacttaggcactcagcaaaaacttccccacctatgtagtataagcgcactcctcttcctatatgccttcttgtcatttctaccgtggcatttcggttaacattggagagtaaacctaagcagaacctctctgaatttgatgggtctgtaaagccatctacagtgagtgagggctgtgatgcatggaaggtttctccaaccctctgatttaattcataatatgctatcgaacaccaaaatgcaggttctgagtaagtaactggctgtaaatccaagctatgattaacaggggaaagagtagtaggagatagttctgctggagagcctgtgtccatactttgattcaactgttggtcacttgtttctccatcttcactgatatatccaggaggtggcgtttctggaatataattactctgtggctcaattcctgctgggaagttagtgttttctggaatggagtgagtatagtcatccagaggcggaagttctgttaggatctcggtgtgtcggggcactaatactggaggcaaaactggtgtctcaactctctgatagtggtaagggtttacacatacttcatcctttttaagattaaaagcatattcgcagttttcaattgccttgagttcatgatgactgtgaagatcaggccagcgccataatcggcaatatataacatgtggcaatccttttcgatgggatacctggagacgaccatcaagagacctggtttgttcagagaagctgtaaaggcctgttgtatcccactgatctatcgtatttggtgtactcagtccccaaatttcagagcaagtgcttggtatggtaacacatttagtattacagttttgagtggtgatggctttctcaagctcatctaatcgtcctgttttctttagcttcttcaccagacttttcactgctttctcacaccacttttcttcctgcccattctgctctcctccgcctgctcctccagacccaccagctgacttcttccatcccagcagtctcttcacaactggcggcgtgaatggcaagatggacgacatgttcttaccaaaggcagcaagccacgctaggaaaacagcctcttgtatcgaacctgcaaggtggcgccaggtcccgccccgtcagatccggggggtccgggaccttttgttccttcctcttccgatgggatggagggggctgggaggggaagaggggaatgggcgattggaggcggaactgaaaacactcccggccgccgtcttcccgccccgcccccaggcccgggcccggccggcggcccgggcgcgcgggagggtaggggaagagaggggaggggaggggaggagagggaaggggaggggagggagcctggccgccgcccgcggggaaggagggggtgaggacgcgcgc

SEQ ID NO: 11475 - RNA, 29906 nt, Homo sapiens
  source 1..29906: mol_type = other RNA
ctgaatagctgggactacaggtgcctgccaccatgcccagctaattttttttttttttttttttgagatggagtcttgcaatgtcacccaggctggagtgcagtggcgcaatctcggctcactgcaacctctgcctcccgggttcatgcgattctcctgcctcagcctcccgagtagctgggattacaggcacacaccaccacacccggctaattttctgcatttttagtacagatggggtttcactatgttggccagactggtctcaaactcgtgacctcatgatccacctgcctcggcctcccaaagtgctgggattacaggcatgagccactgtacccggccccacaatttttttttttttttttttttggagagatgggatcttgctatgttgatcaggctggaaacctgggtcttgaataatggatacatttggaagtgcagagcaaaggccagagagatatccaagccagagagatatccaaggcagaacaaagctcataatttaacaagaaaggtaggcatagataggcctaattatgatgaatgctctcttaccagtataaacaaattacaaagggagtgatgagaagaggcaatgaagtttggggagggaaagaaaagtctgtggtggaggtgataacctgaacttggctttgaggaataaagagttttatatcagggcatcaagagaaggatattcaaggtacttaggaccagaacaggcaaaggcactgaagcaagagagtctggggcaagaatgtctctattgggtcaagactttgacaatattaaagattccattttcttcatatatgcccccctgctgtctttccaataaaggtaagccctgaagcctgacagtcacaggaaaggagagggtgtgtactagagtaacagcacagttgctactcagctgtgaatctcagagcctgcctttattatcttgattattctttggcatctctaggaagatgataagtagtcttcaaagtcagactttactgagaatgagaagggagttctacatgctaagagctccattcacatactaaaagcaaagcttggacaactgaacatgagttttactcctaaccatggataagagaaactgagaatacgatgtgagaagagtctcttcattaggcaggagtggaatgactcccagggcagggagagattgattgagattgcaattgccctgttgggaaataaacggaaacttcaggatgggtatgcgagtcttggagcagcagggttagtcaactactttcctggcatagcctggggaagactgcaagccactcaaaaaagtcctactcatgacttagaggcttacccagtatggcacaggagcactagctcagcattggtggaaggaggtgtctagtcagtctgagaaaatgttggcttcccaaagcttgagcaagatgttcagtacatcccaaagttccaacatcatcccttcccacccactccaaagcccagcagattaacagtcccatagttgggacatggaagctattaaggtagagaccttgagaccaaaggcaatgacagagttgtggtcaggagcagggcatgacagcagtgaacaaaagccagggacccacttacattacccagtagactcagtgacatccagcaaagatggcaggatgagcaccagcagcaggaccgtcaaggacctcagcacatacattagagaaactctttcctgtgtcacctggagatgactgttctcacccactagatgccatcatgaggaagaagctaggaagaacctttgaaaagctgagcatttatccaaagagatggttttaagcctgagataggctatttgaatcgaaagagaacgttatctttgattggcaagtttaaggccatccacctcgtcccacaccttcccaaaaccagatgggatgcatgagaaattgatgtgaaatgaaggaactgtaacttcttttctgcatgatctgagttttaatgtgtgggagctgggaagagggaagaacattgatagaaaatctgaaagcccacagggaatgtggtctaaagcagaggtttaagtcctggctgataatcattttgggttttctgaaaatgcagatcccagtgctccaattccagacctgctaaagcagaatctcacaattgaggccagggaacctacattttagaagctctccttctgactccaatttggaaaccatttatttaaccactagtacaaaaactggccttgaataagacatcacttcctccaagtctgagtacagcacgcaagggcaactgcagcaaatggaggggtgatttagtaaggagggggtgaaaccgaaaatcaacaaggtttgtgtgaactggtctcgacacacttggctgtgaatagcagggatagaaagtagttatggggcttgcaaggacattgtcttaattttcctgttgtcttaacagaggatttactgagcccatgtatgctgtaggaaaaagctagtggtgccagagtttaagttttcagaggaggaataattgacctatgtatgagttctagagaagccttgcagacttacccagggctcagagcacatggcttagtcctgacataaaataccatttttcctctaccacttggctaagaagctgaggaggaactggcagtgagggaggaggttgagaatgaaagttctggagagtcacctaagagacggtaaacacatacctcatgtcttggcttctagagcccggagataagatcagcttcccttgaaaatgttagctcccatgccacatttagtcaagacaacaataacaaaaggctttcttcagggagggcagtggaagtgagtttgagataaaaaggaatttatttatttgcacctatgtattgttcagaagttttaggtcttatgaaaaaaagatttttataaattatacacaattgggtagctttaaaaaataccaaaatatacagtggtcaccctaaaactaacatttttggataatacacttataaattggaaaatgagaaaagatagtctggtataactgcctgaacaacttattaagaacattaacaagtaataacacatattttaatgtaatattgctgactaatttggcacatttaatacacgtccaatatattttctatgtactgtgaaagcttttgggaaaataaagcagcttgtgttacaaaaactgcaacctttcacaaaggttacccacaaaatacttttgcctagccactgcctgtccaacttcagagtggcaccacccttgctattgatctttgtaaccaacgacaattatttcaaaacaattatacaaccctcatttttctttaaaatctttgtcttcctttacttccctgaatacacacgtagtttaccatgacatgggtcttttttttttttttttggagacgtagttttgcactgtcgcccaggctggagtgcagtggcacatctaggctcactgcaacctccacttctcaggttcaagccaatcttctgcctcagcctcccaagtagcgggatcataggcacccaccaatacacccatctaattttttgtatttttagtagagagggggtttcactatgttggccaggctggtctcaaactcctgacctcgtgatcggcccacctcagcctcccaaagtgctgggattacaggcataagccaccgcgcacggcccatgacatgcgtatttctacagcaatgctgtattcccaaatagagttttcttttagagagcctctctctgtgttgacataaatggtgttcagcagtagaacctgaagtaggacacatttcagagagaagtggtgatctcagaatcagtatgcagtactcacaggagccctttgggctctccgcttacatagcttgtctgttctgccccagtgagtcttttctcaggcagagcctcccacttttggcagaggctttttgacttgactttggatttgtcttggttctaagaccactttaataaaggactttacatccctcctgggatgacaaaagactttttgtctttcctggcaagtcctttttgatataaagacaagtgtccctctggtttgagtactctggatttaaaaacaatttttttttagagacagtgtctcactatactgctgaggctggtcttgaactcatgggctcaagcgatcctcctgccttggcctcccaaagtgctgggattacaggcatgggccactgcgcctggctgagtactctggattctgaggcatgccttttctggtaaatttactttgggttcttctgtgtttatattattttttaatctgcatgactgggttaacacttttgggaacactgattttggtttcgtttcgatatggttacatgcatctgtaaatgatttggctcttttcccctgtttctgaacatctcccaagagcaaaaataaacattctaaattttgggcacaggatggctcttttaaagccactagggcaatcgccaccagttaaaacactggtccaaacacctgacttatctgtcaggatttacagaattttctttgctcttaagagattgagaagaaacaaaatggaaattctcaaacattaaggcatgcctgcttttctgggacttcaggtcagctatgtggcttttcctcatgcatgtttttggatcaatgaccatcatagagattgtctatgctttgtctaaactccccaagcttttttattcttagtaccaagagactgcagctatagagttgatatgtagagtcttctaagctctctaattttttttctgcctactttaaatctgctgtttctgccagtgttgagatgaaactcactccttacggcattccagccaagaacaaaaagaaaaaaaaaggtcttaaagggccttaaattaatggctttataaattataatagttccctggcaaccaacacctagaattaagaagtatcccttttaatgtaaatttaggtttgcctaataactgcttagggtgatggaacagttaattaaaggattaatagcctaaaagaactagataaatacgtataaaaattaggctctcaaacaggtcaaaatcttgagctcagggcaataatataaggtatctctggtatagcataaaaattgcttgcctgctatgcaaaggctaaaagaacaaaacaaaaacccctcatccacaactgctaaaatgcttccctgcctgcactgactagtcaaaaaaaccagaatggcaaacaaaagatttgttactaaaaattcaaggccacctggagattgttttttcttatacaattcagccagtcctagctaaaaatgtaagcatttaaatattaacattaaactcatttgaaactgaaaaaagggaaaaaaggggttggggaggtggggtaagaggttttttaaaaatccaaactgctatttaccaaaacttttggttcacagctttcataagattacctattctgcatgtttacccagctgagcaggtcccactttctcagaaatataatttgaatccaataactgtcttttataaaccagcaagcctgtattactatcgtatgactaaaattctaaaatgaaagctatgtttgtgtatgtgtatgtttaggtgtgtttacacatatgtatatatatgttgtatgttgtgtctacgtggtaaaatctggcagttggccacaaatcccttaaggaattctattcatcaaataaatgagtgctaatacaaaatatatagtaattaacacaagtgccttttagttaatataacttaaacatctgataagctggttttaaaataattggtaaatcaaaaataagtgtctttaaaatttttgcctgaatttactactcagttttatatttgtctctgttagactttttaaggtcataaaactataaactcaacttaaaaacagaatgatctttgtataactgtaagttgaactaattttgtattattgacttcagctgtgtcctctgagttactggcaaaatacctacatatttcatttttatggttcttaattgaacacatgatactcacaggtaataaaaatggttaacaggaaaataacttgaaatgactagctatgtctaatatctcagtttttataagtaatctaggaataattgttaaaaatgaattgggggccaggtgcagtggctcacgcctgtaatcctagcactttgggaggccaaggcgggcagatcacgaggtcaggagatcgagatcacggtgaaacctcgtctctactaaaaatacaaaaaattggctgggcgcggtggcgggcgcctgtagtcccagctactcgggaggctgaggcaggagaatggcatgaacccagaaggcggagcttgcagtgagccgagatcacgccactgcactccagcctgggtgacagagcgagactccgtctcaaaaaaaaaaaaaaaaaaaagaattggatggattataaacgggataagcaagggtgagacatggtggtatgcaggtatgcatctatagttccagctactcaggaaacggaggcaggaggattgtgtgagttggagtttgaggctgcagtgtgctacaattgtgcctgtgaacagccactgaactccagcctgggtaacacagcaagacattgtctctaaaaaataaaccaaaagaatgtttttaaaaataggatgttaatgaacttttcatgtaatttgaaatcttataaattaatcttcagtaaatgtctggatcatttccaaaaaaaaacaataaactgctgaaaatattagtttgttcttggcttcctaaattatagaaagactaaatatatttgggcctattaatatacaaagttataaggaaacatgtttctaaaaattataatatggttctcatttataaaatgctgatataacacttcaaaattttgcttcctaggttttcactaaaaattaaggttaataagttaaaatttgaaaatacacaattccatatacaaagtgtacccaaaaaaagatgttttgatgagaaaagttataaggcataaaaattgctttttattgggaaaaaagttgtttaaattcagagtttattagaggttgtttcaaatatggaaacaagacagaaaggaaccactaagtaggaggaggagagaaatatgaaggaagttaatgggtgtgagaatgtacctttggtaaggaaggttacaaaattaacagaataattctgtatgagtcttgcatagtaactttttatcctaaagcaggatgaccagttgtttaaggggaagtataaaacaaagcagaaagtttaagcatgtcactgaaggtctgtgcagatcatgaaatgttcatgaaggatacatttatgaaaggagttgtgtgtaatgaagttggcaataggtcagaatgaaatcataagacattgagcttacatatatacttgtacatatgtatatgtacaataatacagtatattctatacatatgctatatatttgtatatacacgatagtgtaaatgctatacatgcactatacacacacacacacacacacacacacacacacacacacacacacaaaatttggtccccaatgttagaacaaggttctttttaaggatctggtcttaataaaattgaaagaggttttaatttttaattctaaaatcagccatcttctaaaccacagtttaaatttctgccatatttccttctgagatccgtttaatttcccctagattcaggttagaaaggctgtcttttttcatttaagatggtcatttcatttcttgaggtagagttttcttcttgaagatcctgatttatatctcacaagttcaacctttgctgtatcttgctgcaccttatttgtaggtcacacatcattgcctttagctctttctccccttaagaaggtacatctttttgtttggcaggggtgataactcttaactttttcattagctcctgtaacttttttcctctggttctaactcttgctgttataacttgatactgaaatgttctgtagaaggcctagaaaagcaatgttttcctccagtataacttgattctgaattcttggctcttctcatgtttgaattgttccacgcaagcaggaaatttctcgtaatttttccaagagccatgtattctgttcaacatactagctttcttatttacattcctctataaggcgtacactcataaccttggaaatactcttcctgtgtctgattaaattcaagtaccttttcatcagattcaactttcagtatatccaaataggcttcccataagtaaaggcagtcacactgcaagagatttttctttaccattttggcaactggcctaagaaaaattttatgttctatcaagataaattcttgtgtttaagttttttttttgcttgggaaaaatgaagctttgaaaagatggtttttaaatgtatgtaactttctgcattgcttcttaagtcttttgattatcattcttgttaaatattttatagtgacctgtgatcctgtttcgaacttttgacatctttgacaggcttctctaggctcaagttctaaattaagtgtttttgacttaaaattacctttgagttttccacttgggcctctggaaagcctcagagcatgtgtatgccatctggtagagatgttagctaattaggcttctttgatgtattaaattgtatgaaaagcattgtctaatgatgtaatactagacacagttacatttatgagtatgttattgatatgagtgttccaaaattgtacgatgccgttagaaatatgtcatcagtcataattctgattatgctgtttgccacaaaaataaccaaaactctttgtctatttctggttatggtaaactctcatcagatttttaatcatggttattctaagtttttgtaattcccagttattgctttttctctaaaagcatttgcaatcagattcatggaaaagatgctaacacacttttaaatacaggttactaatcactttaataccaatggactaaatattttttcagaacttcaagaaactgatgagtccatgtaactactaattaagatcaaccacaacaaaaaaagttacatgagactaagtaactgaagatgtgtctgtgacttttatttgaagcattattgtttttttacttaaatgttttgttttccatatttaaagaaattctctcatgctatctatagtttacagcaatttggaatacttttgtgaacaaaggtagaaatatttgcttttcctttcttcttgatccctccaatttggaaactattttgagtattcatttgtttttgtttttgagacggagtctcgctctgttgccccagctggaatgcagtggcacgatcttgtttcagtgcaacttctgcctccagggttcaagcaattctgtctcagcctcccaagtagctgggactacaggcatgcaccaccacacccagctaatttttgtattttttagtagagacggtggccggggggaggtttcactatgttggccaggctggtttcaaactcctgacctcaggtgttccacctgtcttggcctcccaaagagctgggattacaggcatgagccactgtgcccagcctatttgtgagtactcttaaggcaatatgatttgcctaagttcaataaaaatcggctctcgttataacaggatacaattggaaacactggttgtattaccaaggctttgattaaaatgtcatatttgagaatgtgtagaatgcctggcttcaatggttctcagcattacactgaattaaaaattatcatttcctggcaggcccaggaaccttaaaactataggtaaaatctaaagtctaccttgacttagcttcttagcctcaaggaggtttttaaatctgagattactgtgaccatactactattcttgcagacaaaatctgataaagtttacaaatctgttttattctgaacatctttggtaaaaatcagggtaactttaagtttctgaagaaagctatatgtacctgttattagatcacagctctgtaccgttttgaaactcctgttatccacctgcagactggatttgctcctgaatcctcctaatttccttcaatatttggctatgactctctaagaaaaaaaactactcccatgctctgaggcctataagctaagatgtgattaatttttaaaggagcaagtctcatgctgatgtatgggtcacacaaaagttcaccataccaaccaatgccatagctagagacattcaaactgcaaaccaggacaaaaagttgatgatttcaggctgtagacatttttcctaagacatcagagcaagaattgtattacaatttgatttattcaattggttgcctgtaagcctaggttcagggctcaaaaccattatgcaaactgggattgtcacattactattaattttgtgtatttcctttttaaactttgtatctgttatttgccaaattttctgcagaaagaagtacaattcctaacagaataatgctagcccagcactttgaggggacaacaaaggactaaggaaaaaaaattggacttaataatagactccaggtggacttagcctaagtgccactcccttaaagcctccctgccctcaaaggtggctaaaagggttttaacactgacttttagttgccaatcactcctgccaatgcaggatgcaggaccagaccaataacccgggaaaggtctattctgtcaccaagggacaatcaaagcctaactacaagatgattcatcatagatactttcggaaaaacatcttcatcaagagagggaaaggtgaaagctgtcagaatcaagagtcatgtttccaaaagccctgacaaatggagccagggaagtccatgaagagagggattttacgcactacctcaaagacccagaagaaaccacgccagcttgcacaaacactattcgcaaccttacacagaaaatacttttgggacatctgcctagaagccgattgtccaaacccgaactggcagcatccttgttattaatccttgtagccaagaataattatttcaagacaattatataatctttatctgtcctttaaaaacctgtcttcctttaccttcctgaatacacacagtttactatggcatgcatattgccttcacaatgccctattcccaaataaacatcattttcttttagaaagcctctgttatttaggttgacagttattacacctgaaaactaaattctagctgatcaataaaattctttggttctactgtatacttttatttggggatatctgcttccaaacacactaaagtacagtatactcaattttaaatatagacagtatatttaaaaaaaacataaaaagtatgtcgaacatttttaatttcaaacaccaaacttaaatagactaataacacagatcttctgtggtccacaaatcatggcaaaaaactttgttttcatatgcccattatggcttgctgactggcttactgcattttagattttccttatgattttagtagctttctctaatggaatgtgctgtgagtgaagcttcaaacattttccattgaatatacacagacatacaaataaagactggaaaaaatatacaccagtcgttttctctggttgttggaatctgggtgattttttaaagtcccatccactgggctgccagtaaaagaccacaaaatatttttgtgtatttacaggaacgtgataatcaaaagttgttgtgggaccattcaagatgagcgtggggaagggaagcccatttaaacatatattcaaggaaaaatatattaagttacctgaacatttgggtagaaatactgagcactgctatggtctgtctcccaaactgtccctcaaatgtatgatgagattttatcttcattgtggtggtgttgagagctggggcctagtgggagatgtttggttcactgaggcagatgcttcatgaatggcttggtgctgctcttgcaatgagttctcactctctcaagactagattagtccccaggagtgggttgttaaaaagagacttgtttggttgttgtgaacaagtgggttgtttgcacgtctgcttcccctctgaccttctccatcaagctatgaagcagcagcaaagcccttgccaaaagccagggccatgcccttgaacttcccagcctgtagaactgtgagcatccttcataagtgaccctgcctcagctatcctgttatagtaacacaaaacagactaagacaggcacacaaaagctgaggactgctgtcgactccactttcaagggctaccaagcacagccacatcaccaaagagaacaattcctgacctccttggaagcagaaacttgactctccgggcaagataactgttgtctttttaaaatttcagtgtcaaagttaaaacatgccttgatcagtcaaccaaattactgctaaaccagtattgggaagcttcctaaagcactccaagctcctaaaaacaggcagcatgaagtaaagcagatagcatctttgcatttaagaagtcccagaaaggttttggaaatggcattaatgtaaatgttcacattaagagaaaacggtttccctgaattgagtgattctttctactttctagtgctgtacaggataggctcagcgtttggagagtgttaacttccagtcatgtgataatggccaggagcaaccacaatgattaacctttagatagaaaacacaatcctttgcttttgtcttccttatgtatattagattaggcttctactcaatgctctgtaagttaaaacatttcaaaccaaataggccactctattaagtcccagcttgagcattcttcagcttctccacattttccattgtttgctggcaaaccagtacagtaacctgttaaatacaaagcaagggtgtggtagattgactgcatttaaggctccaattcttcacccctcctatgttctctcccttggtctaataactctgtagtgcctttccacactgggtttagccatgtggcttgtttctggtgaatgctagttagcatgaagcatgcagacatgaaagggagttatgggattgggcttggctgttgttgccttctacaacctccacaaaaacatgcttgtttaatggaggataggaggcatgtggaaaaatgccaagtccttccaggtgaggccaactccctcatgaacgaggaaagactacaactgctccagagacatctagccgaaatcacttatctaattcataaactgtttattgctgcacaccactgggtttttgtggttgctacgagttacttttgcggcaataattgctccaatatgttctatgtgacatttctgagtttaacatcacatttacaaactttcttagagaaagatttgttattagcaaagaccttcagagtaacctttgcctggtattctagactgtgcagatttagccatctaatactgagtacccacttcaggctgaatgatctctcaagtgctctcatttagttctcataaccaccctaaaaactaacttcctcattttagggaactggaggaaatgaagaactttaaggtagactgatgaaaagatttatctaaagtcacataaattggcacaatcagggtccaaaccccaggcctccgattctgagtcaaactgcattttccattacatcggaaatgaccaaggattaaaattagcagaatgttattctgtccagccattaaaatccaaaaaaaaaatttgttcaaagtaggcaattgagttttcattctattatccaaggtaactgaagtatttgactgtacaggactgcttccttcaagtgttccatccttagcattcttgttaaaaatggcctttaagatattgctattcccagtcaagaaatacccagacaactaaagagactaaaatcatgtaaatcatccatttcccagttgaatcttaaaaaaaaatttatgctcaatacctctctccagccaatcactatgtaaattgtgaattaagacattattacttggtggcaataacggttagaaaaaaagcacatccctctccctctcccgtctccccccgtctcccactttctacggtctcccactttccaccgtctccctctgatgccgagccaaggctggactgtactgccgccatctcggctcactgcaacctccctgcctgattctcctgcctcagcctgccgagtgcctgggattgcagacgcgcgccgccacgcctgactggtttttgtattttttggtggagacggggtttcgccgtgttggccaggctggtctccagctcctgaccgcgcatgatctgcccgcctgggcctcccgaggtgctgggattgcagatggagtctcgctcactcagtgctcaatgttgcccaggctggagtgcagtggcacgatctcggctcgctacaacctccacctcccagccgcctgccttggcctcccaaagtgcggagattgcagcctctgcccggccgccaccccgtctgggaagtgaggagcatctctgcctggctgcccatcgtctgggatgtgaggagcccctcagcccggccgcccagtctgggaagtgaggagcgcctcttcccggccgcccatcgtctgagatgtggggagcgcctctgccccgccgccccgtctgggatgtgaggagtgtctctgcccgaccgccaccccgtctgggaggtgaggagcgtctctgcccggccgccccgtctgagaagtgaggagcccctccgcccagcaaccaccccgtccgggaagtaaggagcgtctccgcccagcagccgccccgtctgggagggaggtggggggcagcccctgctcggccagccgccccgtccgggaggtggggggcaacccccgcccggccagctgccccgttcgggaggtggggggcagcccccggccagcatccaccccgtccgggaggtgggggggcgcctctgcccagccgccccgtctgggaagtgaggagcccctctgcccggccgccaccctgtctgggaggtgtacccaacagctcattgagagcgggccatgatgacgatggcggttttgtcgaatagaaaagggggaaatgtggggaaaggaaagagagatcagattgttgctgtgtctgtgtagaaagaagtagacataggagactccattttgttctgtactaggaaaaattcttctgccttgggatgctgttaatctataaccttacccccaaccccgtgctctctgaaacatgtgctgtgtccactcagggttaaatggattaagggcggtgcaagatgtgctttgttaaacagatgcttgaaggcagcatgctcgttaagagtcatcaccactccttaatctcaagtacccagggacacaaacactgcagaaggccgcagggtcctctgcctaggaaaaccagagacccttgttcacatgtttatctgctgaccttccctccactattgtcctatgaccctgccacatccccctctccgagaaacacccaagaatgatcaataaatactaaaaaaaaaaaaaaaaaaaaaaaaaaagactttagttcaagttgagaccaaagactgtgctattatggggtggagaaaagtatcacaattttggtaatactaggcaagatgtaacctcaagtctccaggcagccccatgagcttccctgtgaatgagaacagaaaaagttcaggagccaccagaggatgttaaggaggcttcctagagaagacgtggcaatgcacctgatggagacgtttaatttcttcactacaaggaatttcaaacttatctaaaaggaaatagaatacaacaaagctcccttacccaatcccaacaaacaaccatcaatgtcctattcattcatacctccatctacttcctctgtcacatactattttgaagcaagtcttacccattgtattttacccataaatgtttcattctgtatctctaaaacattgtctctagacctcagcaaaaaaaaaaaagcacatccacttttacaatggtcacatacaaatggggaaagagtggatataaaaaatatgcacccaccttcaatcaaatgcgatcttttaaagaatataaacaagccagattcttaggtatctctcccttttgtaattttgattctgaaaaaatatttaaagtaatcaattaggtattctaaaagaaggcagttttctaggggtttatttaattataggggggttggggtagagagattaaaaacgggaagcagtgcataggcagtatgaagtagacactttggcaaataaaaactgcaccgtatgacatgtcacatagaaattgttagagactttgaatcctaaaatttagtttaccaaatgtagctttttatgttttatgttttaccaacaaataatttgtatgttaaatttaagcatctgaattccgaaatgataaagaacaggaaaataatgactaagctaacaaccaaactttcagagtataaaattttgtcagtggttttcattttagaattaaaaatttgaatttccctttgcctacaagtctaagtaacttgcagcagcaaattcccccactgacaacttcaaagcatagcaagaatccacagtggtttgcaggccactaattcttttacagatgaaagcattcaattatctctataaaattcaattccttagaatatgtgtttgtgattgacgatgtacatttttaaatgtggtgataacacgttattattcatgatttaaaagttgaaatgaagtagcttgtggttcttgggtaaaacagacactaataagttttttttcaatataaaagagcaacctagacattcctataaaacatttttattccaggtggtaagctggcttaaattttcacttttcagccaggcatgatggctcacgcctgtaattccagcactttgggaggccgaggcaggcaaatcatctgaggtcaggagttcaagaccagcctggcaaacatggtgaaaccctgtctccactaaaaatacaaaaagtagttgggcgtggtggtgtgtgcctgtaatcccagctactcaggaggctaaggcaggagaatcacttgaacccaggaggcgaggctgcagtgagccgagatcgccccactgcaccccagcctgggcaacagagcaagactctgtctccaaaaaaaaaaaaaaaaaattcgtttttctcacagcagcacatttctaaatggcaaaccatttagaagtgagtcatcatttgtattaaaatcttatttacatggtacttatgtagtttgatcaaatactgccacaatatagtttagaggcaagacctctcatgaagaaaaactttacaagatttaaaatcagagcaaatgaatttcttaagttcaagatacgtactctcaatggagaatcgctgttgggcagtggttaaggcctctgatttgctacttattagaaaaatccacatatatacaaaactctgctaaaattccaatggcttctctagatgaatcatctttggctgtgagcaaaaaagttaactaagtttcacttaatacacacacacacactagggtttatatgtagcaacttcctcatcctcattccacaggtagcccgttcttggctgggttatggcttgtaatctcagaaccactgcccccaaatgactgctcagaagcacaatctcactgcaaactatggaacccaaactatacagctatccttggcttttaactccaagctatctaggccttgtgattatatgtgggcttcatagcagaacctaccaggcttgtggttatcaattttctgctcaccatataagcagtagctcaataacaccgtccagttttcatgtatatccagacacacaggtgagagttctgttccaagatctcattttgaccttcttcaaaggtcttctccatctctccaaattgaatgtattcttcaaccctgggcttactgtattctgcccatcttcttcctggaccaaactgttcagaagttaacttctttttcctgtcatcacatctctttcctaaactactttagaacttaaataattttattttcacataacatttagaaaggtgcagaggcagccaacaaaactattgaagacagactgtaaaaactggcaaatccccatctcaaattccatttattctataaccaataaagtcatgcagtttggacgggagcacagtaatacattctgttctcatgtagcttcctaagtatgcttagtctattgttcatttatcactgaatctgttatctgctaagtctgattcaatgttcttgccttctattaatgtgattttaagaattactgcatgtctcactatggcaaaatagcatgacatttgttttacaaaatcagttaaaccaattctacaaatatttccatacctatttattgcagcaaaagataatttttatgtgtaaattagctttttgggtttttctattcctttatttgtaaacttataatttttaggttgggcttactattttgatgagaagggtgaatctgtcaaagggtaagctggataactgtatgttgcaaacatgttcctgaacattcttcacccaaacttagacaaacctggagcttaaaataattacattggatgacatcagtttgatactgatgcctgcttcctgcactaagaggctttcaatctattttgaagagggaaaaacagaatatgccaagtggggagacagcccaaacatagaccttaatacttctctcatactcttcagccatttgatgaacatgtggaattatggatgctagggccattataaaaatctcctgatacagaacagtgtcactacttcaagctaagcagtgacaggcaaagccaggctgaggtgacaatgtagaaggatctcgagtcagccctcaatgttgttgttcaatgttgggaagtcccttttagattatttatacagtggcaggtggtagcaattacagtaaattttcttgggtttcttcctaataaaaaagtgttgataaaactacaccagtcccaaggctattcaatgccacgtaaaatagtgtattttagcatttgaggtccctttttgttgcatactaaagcatgtttaaaatggtttgcagaaaacagtctgctaaccagtactgattcatccacagaactgaattcttgcaaggcacaaaggaagtgtggctgacctaaatatttctcatttttaaaattattcatactgattatatgagattatatcttatctagtatttttcaatggagccttaaaaatgttattttgttaaaagtatatttcagcaaatttcaactttgaagatgtttttgtttacagcatagatcttatgtattagagcgctaatgtagcataggcaaactctgaaataaataaaaatgtataaatagcactgtgcagtgtgtggtgtgcgcctgttgtggggttatattaagtagtataaatttatctcccggggggataggataatcttttatgtaacaccaaattaaaaaaacaaaaacatgtactcttaaaatcatatgtccatatgtgaaatacaatcactttttttggtttccatataatttagggagtgaacaccaaaatgtaatcccatataaaaaaagatcagtttaaataaaaattaaaacaattaaaaattagtcccatagtaacatggtaaacaactcaaatggctttcttttaatgctaggaaaactgtccacctttcaacggtgacagggctgttaacacaggtaagagcaaacaaggtaaaaagtgaaagcacatacagatgatgcacacaaatatatataaaaattgaccagaaatcacaggacatgtaagcaatgttttcttaagcagaactttttttgtactttaaatagactaaaatatttggtgtaggtgggagaaagacatcagtattcaacaattttaacttgaaaaccagctgtaataaagcctcagctcattgtttaataaaaataaaaaaggaaccacatcgtacttttgacaatcatagaacgaaagctcacaaagaacacatttaatatctccatcacagtgcaccaaggatgcagccactaaggacttccagagggaaacaagaacagggtctgcatccatcatattgcattacaaagttaatgccatcagagaaaaaaaatctcacctcacgtgctcaatgttctagctggtaagcaccttatgagtatgaggctacaattgagagaaactgctcagtctgcatcaggacacccaattccttcacttgccattggctgatgcatttaatcattttaacacaacattcacggaaaaatgttaacaacacattctggcttctcgagcagaacagactgggaaatgcagtagacgccagagcatcaaaggccatgtatttcctcacaagaaaagaaatctgcaacaattggtttccttttactatgaaaaatgtaaatttcagattaagtttaaccccataaggacgcatgatttgtacttacatatacacataggttcagaagaacttagctatctagttggcctcttctctgttccattataacatcagttaccttagctggatcactaagtgtgagtctcaccaccatactggtaccttcagctattacctgtgttataaatctcatgttccattcaaagtactaaatgactggatggcacatatcccaataagtatcagaaatgttgacagccatagtgcagctgagtttagaagcaactatgacaacatagggaagtaaggataaatcacaagaacacctaaggtggtcagctccttctggtgtgcctgggacttgttttgagtttagcaaaaactttacaagattaaaaatcagagcaaatgaatttcttaagttcaagatatgtactctcaatggagaatcgcttttgggcagtggttaaggcctctgatgtgctacttatcagaaaaatccacatatatacaaaactctgctaaaagttttgtatccagggaaagtcccgcatccagggaaaccctcaatcccaggcactttagggcagctggtcaccctgagaacactacccactcgttccttaatatcactagagaaaaggtaagaactttcaagggcataacctttaagggcatcagtccccaaaatatttttacatcactagctaatggctagttcctctaagcttgctaaaaggctaggaagtccagaaataccttaaacgtgttaactttaagaagagttggtagtaatcaagcaaattagtgagcagtgtataaaagctcactcttgaaatctgttttcagacaaatcttctaaaggttcttctagctttgtccagttatatggtattttactgtattctctttttgcaattaatccagttttgtatgtcttttctttcttttttaggtgaaaatattctatgccaactgttttccacagtcctgcattatatattaaaacaaaggctgccagctggagacacagccctccgattacaaaggcccagaatgttacttttaactgtgctccaccaggaggtctggccttgggaaaagatggcgaaaggaatattctcagatatgaacattttttattctgcctacaatgctgtgatctagttcaacaactgcagaactgttctcatcttaatcgctgtagtttttctttctttactcttttgtataaaaggttagtgtcacagcttcactatcactaataaaaagatacaaatatgcctttcaagtcagggttggaaaagcaaaactgaggtgtgaggttacactggtctaagaaagtaccaatttgggttctatattttgtcaaacagttgggtttttaaaaaaattcaaaactcatgcatgttacctacttgtcatgtgtgaattatttctcacaattttaattaatctgtgtgtatattagttatataaagcaatggatttccacattcttaaagcaggaacctatattcaccagaaaaggatcctcctgtttctcatcaaattttttttcagctcgaacaatccaagattgggaatagtaagagtggcaaacaaatgttttcttagggacttactgagaaaagaaaaaacttactgggagaacagagacttagtaaaatttctattgctacagacaaatgctaaaaaccagctttataataacagcattataaaggatagaacttaatatagaaccagaaatatggcaagttacctagtgattaacattgtaaaatagtcaaaaactttaaagccacagagaaaggaaaacaattatgaaatggaaaatatataatatttaagtacttttataattctaaaacttcacttttgtccttaaatcaatatattacggatttcattgttcaataaattaccatctttaattaaaaataagtaaatcaaagagcatatttggagaaactaagagctgttaactgtttggagggtaaaagaatacttttctcgaaatttttttgaagaaaaatctaaaagccctctatgttgagttaatacaccttctgacccccatcatcagtggcattattcttccaagggactcttatatctaagcaatggtgaagttctggattcattatggatctcatggcaccaaaccaactggcactgaagttaagttaatatactccagcgagatcacctgtgggtcaaggatggcccagagaatcttggaaaatccatttatattgagcaaagatctgaatcaccttcaatcaggctgtaagatactagaaaatttgaccttgtagtagtatttcccagggtaacttaagcagcaaccttgcaccagaagaagaattaaagagggagcaatctagtattatcaacaacaacaaagttaaccctaagttagtacatcccagaatctgctggatgtataataatttagtaacggggtatatggcagagctttctttgatgttaacaaattttggctgtgattcttagttaccaagttgccaaaaaatggtatattaaatgaactgccaaatggcagattaagaaaattaatgtactccaatggtctgtccatgaaaggaaaatgtacacagacaaattaagaacattttaccaggatctgagatttaaacaatggaacaattgttttaactgttagaatgaccccaactgttaagtttgtctatgagtgtatatgtatatataaattcatacacatatattatttatttccttcttaaaaagactgaggcagttctgctatatatagttagctacaatattcaagataaaacagttcctactcaaaaaattacatgaacacacgagataagttcttatcgtaaatgctatcatgaggctatctagtatagctcatatttcctggttgtaaggctcaaaacacaggaattccactccaagagataatttgcccctcaatccctacaaagtgtagtctaaacaaacaaaatggtaataaaaaattgaaaaggaagatataaaaagaactcaatagcaggattctgactacctctggagaccacacactatcattattctgactgtcttaaatacaacaatccaatatgccccaagatggaaatctggtatcgtagggaaaacattggctgcaactgtcagaaaagttcataatcttaaacataatttatgccatttgccagtcacaaagacatttactgaacagaatttttgagccatttgtaaaattaaaatgattgatcaatttgaatagcaaccttcatgatgaagaaattaggactctaggtatgaaaagcatgttccttttttgttaataagttcaaaggagagaaacattctgatatatgcagataaaaatatggctaggctgggcgcggtggctcatgcctgtaatcccagcactttgggaagccgaggtggacagatcacgaggtcaggagatcgagaccatcctggccaacacggtgaaaccccgtctctactaaaaatacaaaaaattagccgagtgtggtggtgggcgcctgtagtcccagctacttgggaggctgaggcagaagcatggcgtgaacccgggaggcggagcttgcagtgaaccaagatcgcaccactgcactccaggttgggcaacagagcgagactccctctcaaaaaaaaaaaaaaaaaacaaaaaacaaggctaacaagaaagaggataaccagcaagtaccacctggatgtgtgttgtcaggtagaaaggaagaataaaattcaggcaatgaatataatagatttagcaaagtaaagcatatgaaaggaagaaatgtttgatatgtctaagtatcaatgccttcgatcagagtaagaaaaaagtattcattgttcatgtccacagactagatatctaaagagatacttggtgggcaggggcttgggagggaaggcgcaaattggaatgttcagcttttaaagtaaagactgtacatgaagacatattttatgtacagtgaagattgtcttgtgttactttatatcccaacataaacctacgccaccctcagacgaagagggtatctaacactgaataaatgctgaacctatttagtagttaaagaaaaaagagaaggatcttaaaggtatatatgggaagcttttaagaggtagagaaaccaactgggtatatattttcttttatttgatttcaactagcaagagactaagactgatgtttgtttgtttgttttaccttcaaagtcttagtcttaaattgacaagggcacaaaaaaagtgaaattaaaataattttaacaaaagggaaagcatttgacagtgtttaaaagacagacaaatcaagcaaaactcaatgtggcttaaggtaaaaaatacaactaggtattaaacaatttgtaaaaacttacaaagaaaatttagctttcaagaaaaattaggcagatttccttctgccaaagtgacaggtcctgaggaaaaaaaacacaacctctacaagaccaagcacagctcaagggtcagggccccgtcctagtcatctttttattattcaatatccatcacagtggctgggcaaacaacaggcatcaataaatgtttactaactgaatgtgtattataaggtataatcggtataactgatatagctcaaatctaatcatgaaagcttctttaaagtaggataaaaagagcacaatcagcggtattccagaaggtaggcctaaatccagttatatttttctaatcgttgaccagtggttataaagactttctgagcttctttttaaagcaatgaaactctttccaaaagaaaccccatgcagttcttcagtacagaataaatatgccactaagtcagtgagaactccaacagcctcccctaagccagcccccaaggtgtctctgtggaacctactggaaaaaatattactcatcttagaaatgtgatagaaagcatggccattcggttctcaggtcatcattcctagaaaattaacagtattgtgaagaataaatcctaagtaatgttgctaatttaaataaagacaaaaattcaacaaagaggggattctatcacttagaaaaatgaaaaccacacctataaatggggggaggggcagaaaacaaaaaaaaaatcaggccacagtagataaaatacaaaaaacatcatctcgttaaaaagcatcaaacacattcacacaaatgtaattacaaccaggaagtaaactgctcaacaggtataactgctcaataggtgttttcaaagagttgagtcccaatttcatactgtacagaaaaatcgcatcagaactgtagagatgcgctccactactgaaacagcatagtaggcactgcttgacctaacacagtaatgcaagagtaaccaccaagatcaggaccttctaccactttcagagttgttttctgcccctacaactgttccctaacaccattacaagttctcaagtaagaaaaagaagggcagaggctccactgagtatctcctacaggcctgatagtggtattacctaggacatttactctgctcacaagatgggtagtggaagacataattactggacagcacaaagtctggaagcaagcagcagggcactaaaacagtgagagcttacacaacaaaagcttgttaaattaagtagtactgatgtggtgcaaatgaaatttttacagcaaaggttgaggaaggagatatgttagtgagaatcacatgaagcagactatcacaaaataaggccaccttcaaaatgttatgaactgtagaaccattctgatcttcaagtttggatttgtatagaggtttctgtataaagcattaatacctaatcaggagtttcctttagtgtgaacctttttgcatttgatgctattctctttgccaggaatgcttatctcccctggctcctcacttggcttgcttctttaatgtcaggtgttagctcatgcatcctttccttagaggctttccttgatgtcctacctgaagcatcccatctgttattctccagtacagtaccctgtttatctccttcatagacaagtaagataattaagggttagtgtaactgctgtctcagcaaaggcaggaactgtagttgtcttgttcacctttacccaaagactaagaaaagttcctggtacaaacaggtgaacaataaatatttgttgaatgaataaaaaattactataccaaatttacatgaacacatacatatacacacaaatataggaaaatggggagtacccaatagaaaaccaccaaatgttgaaagtattgaaaatgatacctatagagacaggtggatatgatttcaaagaacaagtaccaaagacagcttcaaaaatatgaaaatttatgaaaagacgaccaggagtggttattttccatttctactaagatgcaaacaagaagaaatgtttaaactgcaatgagtcaacatcagacataataattatttgctgcagaatgaactagcaacagagtttcggaaatctcctctcactacagagcatgaaatattgtcaatcacaaaaccaggatcagttaagaacagctcagactgcaggtaacttataagctaaaaaacttgctaaataaatggcttttcccccaatttttaaaattctgaattcataattatgtgtagaataacaatcaatttataaactgaatacaacatactttaaaaacagatggcccatatctgctgatcctacctcagcatcacttttctaggtattttgcagaaacaattacatttacaaaaggcccatttcataatgcaatctggttactaaaccaaatcaaactactcgaagagcagaaggtctgctgttgaaatattgtaaaatacctttggaaaaacggtatttatagattagcttttttaaaaagggataaatatgtggaagtaattctagcatatccctgaaaataattatactgccacctatgcattttttatgaggtggaaggataaatcaacagactgctagattatacaagccaattattcctgttgaaatttgggcataagacaaagggactttctccatatgaattcttactgtatcccagaattaactggtgccagcagtatcaatgcaactattactggtgatgatgtcatgttatgctgttttgattatgaggacaaaaatgggaatggaaaaaagaggcttggaaaggttttcagtatggtttccttataataagatttagcagttaaaaaaaaaaacaaaaaaaaacaaaaaaccacaaaaagaatgactgtttaagccccactgaacacattaaggtcaaggatttcaaaagttaatccacttttcttcccccaagagtttatttttggtaaaaggcagaaaaattagtttttctacaggaaaatctgcttctaaataatttgaaaatcttgatatatattatatattaaaaaagacacacaaaaataacagagaagtgggaataacagattaggtactgcaactttataaaggtttgcctagatcaagaagcagcgcacacacacacctcatctatgcaaactaaaaatgtatataaacagcacaatactgtgatactggatcatgatacattacctgtacacataactactactgttattaataaacctttgggacactcagttttatgcccaataagacatcattaagtctttaaaatcttctcttcctctttaatgggagagtatttctagacactaattttcccatctaatattcaaatataggaaacagattccacaaggtgctttaattgatgagacctcaagtgctgttttctctcttgaacttttggatagtaaacagtccatagggaccacacacaatgctatgacagaagagttgttacattaagtcttttcatgggacttgattggtgaagctttatgacatgcttgagcaacgcactgaaggggatcccatctgagttaatactttgtccaaccactgtagaggtccattcagatgaagttcaatccagcaaggagtacttgttaccgtctgccttcggtattctgctccccaccctttcacaaaactcattcttatggtgcacattctagttagctgatagacggcttcaaaaccctgattaacagactgagccagaagagcagcaaattcctggttgttgaagatcttcagattacagcctggtggaattttacacactgttgcagggtgccagccatatctctgattacaattggggctctgcacaaagattgcactatcacttaggcactcagcaaaaacttccccacctatgtagtataagcgcactcctcttcctatatgccttcttgtcatttctaccgtggcatttcggttaacattggagagtaaacctaagcagaacctctctgaatttgatgggtctgtaaagccatctacagtgagtgagggctgtgatgcatggaaggtttctccaaccctctgatttaattcataatatgctatcgaacaccaaaatgcaggttctgagtaagtaactggctgtaaatccaagctatgattaacaggggaaagagtagtaggagatagttctgctggagagcctgtgtccatactttgattcaactgttggtcacttgtttctccatcttcactgatatatccaggaggtggcgtttctggaatataattactctgtggctcaattcctgctgggaagttagtgttttctggaatggagtgagtatagtcatccagaggcggaagttctgttaggatctcggtgtgtcggggcactaatactggaggcaaaactggtgtctcaactctctgatagtggtaagggtttacacatacttcatcctttttaagattaaaagcatattcgcagttttcaattgccttgagttcatgatgactgtgaagatcaggccagcgccataatcggcaatatataacatgtggcaatccttttcgatgggatacctggagacgaccatcaagagaccttggtatggtaacacatttagtattacagttttgagtggtgatggctttctcaagctcatctaatcgtcctgttttctttagcttcttcaccagacttttcactgctttctcacaccacttttcttcctgcccattctgctctcctccgcctgctcctccagacccaccagctgacttcttccatcccagcagtctcttcacaactggcggcgtgaatggcaagatggacgacatgttcttaccaaaggcagcaagccacgctaggaaaacagcctcttgtatcgaacctcccggcggctggcgggctgctggctggcgagctgcttctccgccgccgcggccgcgcgggtagacccgcct

SEQ ID NO: 11476 - RNA, 4885 nt, Homo sapiens
  source 1..4885: mol_type = other RNA
ctgaatagctgggactacaggtgcctgccaccatgcccggctaatttaagtattttcagcagagacagggtttcaccatattggtcaggctggtctcaaactcctgacctcaggcgatccacccacctcagcctcccaaagtgctgggattacaggcgtgagccctgcgcccggccagctctccttacatcttgatttcaatcctataaatgggaaatggtagggagcactgtctagtctactgtgggatttctagttgtcataacaataagaaccatataaacaacgcccacctggtaaacattagggtggcccaggaactctgcagcagtcactgagcacattccaaagagcggatgttaaccccccaaccccgtattttaaagggctagcttcagtctggctgccaatggttacattttttcttccccaccttgtgtttagcctccccttctgtgtccaacctcctccacttctcaatgaccccaagggcctctgtaagtgcaggattctacccaaaaccctcccaattccaaagggtgggccttggcataaagaggcatcattccagggtgctacacggtggcttctgagggaagaccaagaaggctgaacctgttgtatttggtaatgaattttgttttctcctgggttgggtgagcaccttaggagcttactgtggaagcagagtcctagcgaaaataagactggcattgataggatgtcttgtatcatcaaaatgcttaacaggtccatgaaacatcctagcattgctgtgagagtggttccaaggtttctatgaatggtggaaacagacacaaacgaaatgtgggaagaagctttgggaagaccaagaatgaaaaaaagggaaaagaacctaacactcaatgcaatgctacttaaggagaaaaatacataaaccgttcttcaagctttaggtccaaaacaatgttctctcttaagagggtggtttgcaaacagggaccatgagataatttacaatcaaatcatttcagatattgaatgatgattctgaaacacgcattctatttccatcaatgtgaggtttatttccatagaaacggtgaaaaaagtaggccaaacccagcagtatggcttctaaaaggaatagcagctgtggttctggccagccatggaaagcactggttttgtaactactatagtaaagagctctgactgaagggaaatagaaagtttcaactcaaagaaagggcatggaaagtatctgagaactttcctggctgtttcttacaaagccatggagaaaaaatcatctcctgtgcaccctgctcttcacaatgccacagtaaagtcgaattcaccacctgcgaaacagctgcctcctgtaggctggcctcagaggaagcacacatgctccatcagttgcaacaaggcgaaagtcagaagagtgtgaaagtgtcaggcccagtgctcccggaaaatgaacccggaaacactcagtgaggcaccaccggtgtgagaaagaagagacaggtgtcttctccaatgggcacaagtatgtcatgcttagaaaagcagaacacaggatgaaacaaaacatatttatttgcaaagaaagatcatgtttaaattgtacctgtgtttaaaaatggcctctttgatgggttataaaagtgcaggcaggttttatgaaacacgcactttgcctctcttctatccttttgtgggaagcaggcagatgctggctggaggacatttgagagctcggagctgaggctcatcacagccaaatccctcactcaccaagtgagcggagctgccactgacgcttctccactcccgcagaatctactattgagcactgggccccctgaggacaggatgtgaccctggctggcatgattcattcaacccgttcatcttggaattcttttgcagaaaaaaaaaaagtgacacttctatggctaaagatttccttaaagaagaagaaacatcagaacgaacctttgtgctgtgtgaaatgagggaacaaaagattactttcagtgagttgatatctgtaagctaatcaactgggtactggcctcttgttagaggaaaaaaaagtccaacttggaaaccattaccacaggaaaaaacaatgactatgttgttcattcctgttggtcacttgggtagtctaagaagtaggacatatatgtctgtaagccctttaaaatacacatcttttcttttttcttctcactatgtaaaacacatatatattatcctaaagtcacttgaaaaacacagactgcttacaatcaatagaagataccagtaagatgcaagaaaatgagcattttacagacagacctttgataggctttaaagtgaatcgtttttatttaaaacagggatccatcagaggtggtgaactatcaaggtcaaggttctagagcatggcacagatgaaaggtaatactcaccagcacctcacatgggactcagtgacaatgtcagcaacacaccatggaaggagaacaaacccgatgtaaaaggcacctagctggggagaagctgtggtgttcactgcctctctagcaggtttgcttttgtgcactgtggctaagtctggatgaataatattgggaagggaataatcggaagcgaggctcctatgcaggcagctaccctctcctgattggtgtatactcgccatgtggtaggaggtcttacaggagactgaggttaccaaacaggaatacaacacctctctcccttttctgctctagaaggaaggggaacccttcccccagtatcaatttcagcagcggcttctaaaggctgttaaaaagcatcctaacttaaaaacaaataacaacagtaaccaaataaaagacagaaaagtggcctgaacttaaatcaatcaatggaaaggtagattcataaaaataaaataaaaactggtgaccagtccattaaccatggggttaatgcctcgtctgaaggaagatgtttacgctgcatccacgatccagcaggcgcggagctgctcttggcaactgtgaatgaatagctaccgtttcccttcaacacaccgcgctgccaccggtgaccgcatgtcaagtgctgaagttagaagagaccccacgttggcaaaggccccccaggcgatgatctgcctgacgcggccaggtctgtgggaaacaagacttacgatctcaaataatgacccccaagtgccctcgcctcttcctgcttgccctgtgcgcctcgacctcctcacggggagttccaaatgagttccatttccctctcagttctaggcactctggaacatctttgattaaccagggtttttcatttctttccaacgccattggtgacttttgacttggaatgccgattccttctcctggaagaatggctttcgttgttgcctgcatgcttgggtgggctgtcttcagaaccttttgtccctttcctgtgatgccaggagatctctggactgtaggtgccatcttcacactccgagtaggtcttttctcggtgaccatagtgttctgcataccaaatcatgccgtacagacagaggaaagtggtgaaagccacgcaaagaagccaaagcacaacatagagtatttgggtcttagagaagagatcttgtccaaattttatgcaaacaatggcctccaggaaaccaatgaccccaaacacccagcattgtgttcctacgcgcttgcactgtgtgtcggtgaggtaagcgtagtactgtctcactgtgggagctgtgatgccaccaataaagagaattctaccccaacttaatggatgactggcttggaacacaaagatatgcttcaagaagaaggtattcaactcagtcagctgccagatgatcatgaaaaggtacactccagctactctctgaaaagaagatttggggtcaaaccatcgaacataggtccagctagcaggagtgaactgcagaacagctctcttgatcttcccggtggtggtatgaatgtccttgaagcttgcccagtggtaagtcctcatctctaaaaaccggcaaacgaccatgcccagccaaatgccaccgccattgcacaacaggatgtccagaatgacttgatcccaccagcactcggcaaaattggggaggagatgcatgaagaagagctcagtcagctcccaggtaatactgattgtccagcagagaccgtaactacggatcagcaaggccttcatggcccagccccagaaatgtccaaatgcaaaaatatcaaagtggctgataatcctctcccaggtgatcacatggcagttcacagcatactccatgacatctgcttcccttgtggcgtatcgaagatttggatctagccaatacattagagatttaacctgctcgaaattcaggaagagtaggaataccaggaacaggaagtagagcacactgagtccaaaaaccattcgccataaggctggatgaggtcgagtgaacggaccattggggaaagctaacacactgatgataagaaagaagaaaataacagagaggatgcctctccagatgttgtcttctggaacagagtcatccctggtaaaggcgaagtacatgaggctgacgatggtgaagctgagcagggtgatggtatgcggccggtagaagaagtcaatggtgatgtcctccacttgctgctcgttgatcatccggaaatgcattttgtagttcacatcatccttgcttagggtccggctccccacgcaggacgccatggcccgcctccccgtcctgccgcggtggcggcggccccagcccgagaaggccgggaccccgggggtgactagccacagtaggctaatagccggacggcaaagccgggtctggcgcccagcaaaggctgggagcagaggg

SEQ ID NO: 11477 - RNA, 4715 nt, Homo sapiens
  source 1..4715: mol_type = other RNA
ctgaatagctgggactacaggtgcctgccaccatgcccggctaatttaagtattttcagcagagacagggtttcaccatattggtcaggctggtctcaaactcctgacctcaggcgatccacccacctcagcctcccaaagtgctgggattacaggcgtgagccctgcgcccggccagctctccttacatcttgatttcaatcctataaatgggaaatggtagggagcactgtctagtctactgtgggatttctagttgtcataacaataagaaccatataaacaacgcccacctggtaaacattagggtggcccaggaactctgcagcagtcactgagcacattccaaagagcggatgttaaccccccaaccccgtattttaaagggctagcttcagtctggctgccaatggttacattttttcttccccaccttgtgtttagcctccccttctgtgtccaacctcctccacttctcaatgaccccaagggcctctgtaagtgcaggattctacccaaaaccctcccaattccaaagggtgggccttggcataaagaggcatcattccagggtgctacacggtggcttctgagggaagaccaagaaggctgaacctgttgtatttggtaatgaattttgttttctcctgggttgggtgagcaccttaggagcttactgtggaagcagagtcctagcgaaaataagactggcattgataggatgtcttgtatcatcaaaatgcttaacaggtccatgaaacatcctagcattgctgtgagagtggttccaaggtttctatgaatggtggaaacagacacaaacgaaatgtgggaagaagctttgggaagaccaagaatgaaaaaaagggaaaagaacctaacactcaatgcaatgctacttaaggagaaaaatacataaaccgttcttcaagctttaggtccaaaacaatgttctctcttaagagggtggtttgcaaacagggaccatgagataatttacaatcaaatcatttcagatattgaatgatgattctgaaacacgcattctatttccatcaatgtgaggtttatttccatagaaacggtgaaaaaagtaggccaaacccagcagtatggcttctaaaaggaatagcagctgtggttctggccagccatggaaagcactggttttgtaactactatagtaaagagctctgactgaagggaaatagaaagtttcaactcaaagaaagggcatggaaagtatctgagaactttcctggctgtttcttacaaagccatggagaaaaaatcatctcctgtgcaccctgctcttcacaatgccacagtaaagtcgaattcaccacctgcgaaacagctgcctcctgtaggctggcctcagaggaagcacacatgctccatcagttgcaacaaggcgaaagtcagaagagtgtgaaagtgtcaggcccagtgctcccggaaaatgaacccggaaacactcagtgaggcaccaccggtgtgagaaagaagagacaggtgtcttctccaatgggcacaagtatgtcatgcttagaaaagcagaacacaggatgaaacaaaacatatttatttgcaaagaaagatcatgtttaaattgtacctgtgtttaaaaatggcctctttgatgggttataaaagtgcaggcaggttttatgaaacacgcactttgcctctcttctatccttttgtgggaagcaggcagatgctggctggaggacatttgagagctcggagctgaggctcatcacagccaaatccctcactcaccaagtgagcggagctgccactgacgcttctccactcccgcagaatctactattgagcactgggccccctgaggacaggatgtgaccctggctggcatgattcattcaacccgttcatcttggaattcttttgcagaaaaaaaaaaagtgacacttctatggctaaagatttccttaaagaagaagaaacatcagaacgaacctttgtgctgtgtgaaatgagggaacaaaagattactttcagtgagttgatatctgtaagctaatcaactgggtactggcctcttgttagaggaaaaaaaagtccaacttggaaaccattaccacaggaaaaaacaatgactatgttgttcattcctgttggtcacttgggtagtctaagaagtaggacatatatgtctgtaagccctttaaaatacacatcttttcttttttcttctcactatgtaaaacacatatatattatcctaaagtcacttgaaaaacacagactgcttacaatcaatagaagataccagtaagatgcaagaaaatgagcattttacagacagacctttgataggctttaaagtgaatcgtttttatttaaaacagggatccatcagaggtggtgaactatcaaggtcaaggttctagagcatggcacagatgaaaggtaatactcaccagcacctcacatgggactcagtgacaatgtcagcaacacaccatggaaggagaacaaacccgatgtaaaaggcacctagctggggagaagctgtggtgttcactgcctctctagcaggtttgcttttgtgcactgtggctaagtctggatgaataatattgggaagggaataatcggaagcgaggctcctatgcaggcagctaccctctcctgattggtgtatactcgccatgtggtaggaggtcttacaggagactgaggttaccaaacaggaatacaacacctctctcccttttctgctctagaaggaaggggaacccttcccccagtatcaatttcagcagcggcttctaaaggctgttaaaaagcatcctaacttaaaaacaaataacaacagtaaccaaataaaagacagaaaagtggcctgaacttaaatcaatcaatggaaaggtagattcataaaaataaaataaaaactggtgaccagtccattaaccatggggttaatgcctcgtctgaaggaagatgtttacgctgcatccacgatccagcaggcgcggagctgctcttggcaactgtgaatgaatagctaccgtttcccttcaacacaccgcgctgccaccggtgaccgcatgtcaagtgctgaagttagaagagaccccacgttggcaaaggccccccaggcgatgatctgcctgacgcggccaggtctgtgggaaacaagacttacgatctcaaataatgacccccaagtgccctcgcctcttcctgcttgccctgtgcgcctcgacctcctcacggggagttccaaatgagttccatttccctctcagttctaggcactctggaacatctttgattaaccagggtttttcatttctttccaacgccattggtgacttttgacttggaatgccgattccttctcctggaagaatggctttcgttgttgcctgcatgcttgggtgggctgtcttcagaaccttttgtccctttcctgtgatgccaggagatctctggactgtaggtgccatcttcacactccgagtaggtcttttctcggtgaccatagtgttctgcataccaaatcatgccgtacagacagaggaaagtggtgaaagccacgcaaagaagccaaagcacaacatagagtatttgggtcttagagaagagatcttgtccaaattttatgcaaacaatggcctccaggaaaccaatgaccccaaacacccagcattgtgttcctacgcgcttgcactgtgtgtcggtgaggtaagcgtagtactgtctcactgtgggagctgtgatgccaccaataaagagaattctaccccaacttaatggatgactggcttggaacacaaagatatgcttcaagaagaaggtattcaactcagtcagctgccagatgatcatgaaaaggtacactccagctactctctgaaaagaagatttggggtcaaaccatcgaacataggtccagctagcaggagtgaactgcagaacagctctcttgatcttcccggtggtggtatgaatgtccttgaagcttgcccagtggtaagtcctcatctctaaaaaccggcaaacgaccatgcccagccaaatgccaccgccattgcacaacaggatgtccagaatgacttgatcccaccagcactcggcaaaattggggaggagatgcatgaagaagagctcagtcagctcccaggtaatactgattgtccagcagagaccgtaactacggatcagcaaggccttcatggcccagccccagaaatgtccaaatgcaaaaatatcaaagtggctgataatcctctcccaggtgatcacatggcagttcacagcatactccattggggaaagctaacacactgatgataagaaagaagaaaataacagagaggatgcctctccagatgttgtcttctggaacagagtcatccctggtaaaggcgaagtacatgaggctgacgatggtgaagctgagcagggtgatggtatgcggccggtagaagaagtcaatggtgatgtcctccacttgctgctcgttgatcatccggaaatgcattttgtagttcacatcatccttgcttagggtccggctccccacgcaggacgccatggcccgcctccccgtcctgccgcggtggcggcggccccagcccgagaaggccgggaccccgggggtgactagccacagtaggctaatagccggacggcaaagccgggtctggcgcccagcaaaggctgggagcagaggg

SEQ ID NO: 11478 - RNA, 2669 nt, Homo sapiens
  source 1..2669: mol_type = other RNA
ctgaatagctgggactacaggtgcctgccaccatgccctgctaatttttgtatttttagtagagacagggtttcaccatattggtcaggctggtctcaaactcctgacctcaggtgatccacctgccttggcctcccaaagtgctgggattacaggcatgagctaccatgcctggcccctgagatctttaaaatcatggagctatattctagctggggtcaatagactgaaatgtcagccccatacctggcatataggaaggacatttcccctcctcccacttgctctgcttattatatgtaataggggtgtggaggaggcaagggagctgaattgggggcagataggggaacagtttggagatttatacaatctttgtgaatatcttcctttttttcttcgagttaggttagactaggacattgcctgcttccagcagcaccaccaggactgctgctggaaggacttcagagggtcaagaaaattctccaaagatttttgtgtctcaggcgatcccagcctcctctgtatttccagggacctgaggttacaggtggggattatcagaatatcagagagggtcctcgcccaaacaacaggatgccccaaactgaaggcttgtcatttatctctgaaagaggcaagtcaacaccttaatcctcatcatagcatagtcctcggtcctcagtggcaagggtgacttgaaagtggggcctttcatagctccagagccaaggaggccttgacaattaggcagagagaagacctggatgtccatcccatctgataccctgacttcccaagagaacaacccattcttctcagatttctcccaagtccctcattgctgggcctggaggctcgctttggctcctgtggtctctggaggatgcaggcatgaagcctgacctgacttgtactgaccctgtcccaggccttttgtgtctcgcctacctggctactcctcgtggccctacctatccaacagactgtgtgcaggtgggcaaggccaggctgtcttccaggagtcagtcccaacactcatcagcaaaaaggggtccgtgtctaggtgtctgggactggtttaagtaagaagagagtgccaagacccctctctctcttccagggagtgaactgatttctgacttgagttgtttaaattgggaagaggcctcatcagcaatcagagaggtctagatctctggaatctggccacggagtgattttcccatcagcctctgtctcggtgactgaggatctcggggcttcttcttttgcctctgacccaaggcccctcacacacttcttccagtgagccaggcagtgatgggcagaggagcggatctctccactccgtagagcatagatgacagggttgaccatggagttgatgaggcacagcatggagcagaaagcaaaggccttcttgacctggtcactgagcgtagtggccaggctgtgggccatgagggccagcactgggaaccaacagatgaggagcacagccaacactagccctagggtcttggccaacctcacatccagcctcattcgggccattcctggcacctgcctgtcctggtggccagacaagctggccacatgctgatgggccttccagagaacatgcccataggtgtagatgattccggaaaagaggaaggcgatgaacaggagccagctcagcaggtagtcattggggatcagtgggaaaagctcagagcagggcctgggacagcaagtccatcccatgaggggcaggtaggagactagtgctgagaggacccacatgatgcccagggtcaccagtgcccttccacgggtgagcagagctttgtaggaaggtggatagcgcaggcagaggtatcggtcaatggcggtcagcaggaggctacccacagaggctgtgaaggtcatagtcacgctgccaatcttcagcaggaagacagccttggaatccacaccatggaaaacatggaaattcacaaagctgcatgcaaagaccacactggccaggaagtcagccccagccaagctgccaatgaacaggtatgagggcttccggcggagttggtgggaggacaggatcagatagagcacagccacgttctccagggcacttagcaggcccagaagagtgcacaacacagcaacagctgtcttctggggaccactcaggatcatgtaatccttcatagggttggaatccaagccatccttggagccattggctatctctgtcacccagcattcctccatggggtgggcccttcagattccactgagcttgtctagaaggctttgctatgccattctccttgagatgccaaatgggctgatgacctccatcatagcttcttaccctgggtccatgggtaggcttggatgggagtatcggtcctttcgaggcatatttaagactttatgtctgtgcatgttttggttggggtagaaggattcacactttttatcagtgtgccagcagagttctgaatattaagaatcaccgatgcatgcaaaaacattttgtgacctgatgctgtacagatgtaagagtaaaagagaagcgggagtctttctgaacctattctgggctgcctgattaaaaaagaaaaaaggccaggcgcggtggctcacgcctgtaatcccagcactttgggaggccgagg

SEQ ID NO: 11479 - RNA, 3361 nt, Homo sapiens
  source 1..3361: mol_type = other RNA
ctgaatagctgggactacaggtgcctgccaccatgccctgctaatttttgtatttttagtagagacagggtttcaccatattggtcaggctggtctcaaactcctgacctcaggtgatccacctgccttggcctcccaaagtgctgggattacaggcatgagctaccatgcctggcccctgagatctttaaaatcatggagctatattctagctggggtcaatagactgaaatgtcagccccatacctggcatataggaaggacatttcccctcctcccacttgctctgcttattatatgtaataggggtgtggaggaggcaagggagctgaattgggggcagataggggaacagtttggagatttatacaatctttgtgaatatcttcctttttttcttcgagttaggttagactaggacattgcctgcttccagcagcaccaccaggactgctgctggaaggacttcagagggtcaagaaaattctccaaagatttttgtgtctcaggcgatcccagcctcctctgtatttccagggacctgaggttacaggtggggattatcagaatatcagagagggtcctcgcccaaacaacaggatgccccaaactgaaggcttgtcatttatctctgaaagaggcaagtcaacaccttaatcctcatcatagcatagtcctcggtcctcagtggcaagggtgacttgaaagtggggcctttcatagctccagagccaaggaggccttgacaattaggcagagagaagacctggatgtccatcccatctgataccctgacttcccaagagaacaacccattcttctcagatttctcccaagtccctcattgctgggcctggaggctcgctttggctcctgtggtctctggaggatgcaggcatgaagcctgacctgacttgtactgaccctgtcccaggccttttgtgtctcgcctacctggctactcctcgtggccctacctatccaacagactgtgtgcaggtgggcaaggccaggctgtcttccaggagtcagtcccaacactcatcagcaaaaaggggtccgtgtctaggtgtctgggactggtttaagtaagaagagagtgccaagacccctctctctcttccagggagtgaactgatttctgacttgagttgtttaaattgggaagaggcctcatcagcaatcagagaggtctagatctctggaatctggccacggagtgattttcccatcagcctctgtctcggtgactgaggatctcggggcttcttcttttgcctctgacccaaggcccctcacacacttcttccagtgagccaggcagtgatgggcagaggagcggatctctccactccgtagagcatagatgacagggttgaccatggagttgatgaggcacagcatggagcagaaagcaaaggccttcttgacctggtcactgagcgtagtggccaggctgtgggccatgagggccagcactgggaaccaacagatgaggagcacagccaacactagccctagggtcttggccaacctcacatccagcctcattcgggccattcctggcacctgcctgtcctggtggccagacaagctggccacatgctgatgggccttccagagaacatgcccataggtgtagatgattccggaaaagaggaaggcgatgaacaggagccagctcagcaggtagtcattggggatcagtgggaaaagctcagagcagggcctgggacagcaagtccatcccatgaggggcaggtaggagactagtgctgagaggacccacatgatgcccagggtcaccagtgcccttccacgggtgagcagagctttgtaggaaggtggatagcgcaggcagaggtatcggtcaatggcggtcagcaggaggctacccacagaggctgtgaaggtcatagtcacgctgccaatcttcagcaggaagacagccttggaatccacaccatggaaaacatggaaattcacaaagctgcatgcaaagaccacactggccaggaagtcagccccagccaagctgccaatgaacaggtatgagggcttccggcggagttggtgggaggacaggatcagatagagcacagccacgttctccagggcacttagcaggcccagaagagtgcacaacacagcaacagctgtcttctggggaccactcaggatcatgtaatccttcatagggttggaatccaagccatccttggagccattggctatctctgtcacccagcattcctccatggggtgggcccttcagattccactgagcttgtctagaaggctttgctgggaggctgaggtcaaaggattacttcagcccaggtggtccagtgtgcagtgatctatgattgtgccaccacactccagtgtgggtgacagaatgagacctcaatagtagacagagaaatgtgtttcactcccatcagatcggtaaaaaagtaaggctgacaatactgagtgctggagaaggcgtggagccaaaagaactctcattgcgatgggggtgtaagttgacacagacactttgaagagcagcttggcaaaatctggtgaagttgacgatacatcaattgcagtcccgggaatacgttctggaggaactcctgcaggtgcgtccagggaggcatgtacaagaatgttctctttggcatttttgaaatagaagaacaattctaaatgtccatcaacccatgtagaattcagcctagaagagggatgctggggctgatggaggctggcttcaggtctcatctaggcctggcatggccaccaacatgtgtggttattatccaaagtagataagggaaagaaattcaggcatttggatgcaggtcttaacaagccagcatctgacaatgggacacacagagcaacgggaaacccagctcactgtcttccctttggacagctataaatcccttttggagtcagaatctctggcttctagacagggcctttttccagggtgaagactgtgtctatgccattctccttgagatgccaaatgggctgatgacctccatcatagcttcttaccctgggtccatgggtaggcttggatgggagtatcggtcctttcgaggcatatttaagactttatgtctgtgcatgttttggttggggtagaaggattcacactttttatcagtgtgccagcagagttctgaatattaagaatcaccgatgcatgcaaaaacattttgtgacctgatgctgtacagatgtaagagtaaaagagaagcgggagtctttctgaacctattctgggctgcctgattaaaaaagaaaaaaggccaggcgcggtggctcacgcctgtaatcccagcactttgggaggccgagg

SEQ ID NO: 11480 - RNA, 2421 nt, Homo sapiens
  source 1..2421: mol_type = other RNA
ctgaatagctgggactacaggtgcctgccaccatgccctgctaatttttgtatttttagtagagacagggtttcaccatattggtcaggctggtctcaaactcctgacctcaggtgatccacctgccttggcctcccaaagtgctgggattacaggcatgagctaccatgcctggcccctgagatctttaaaatcatggagctatattctagctggggtcaatagactgaaatgtcagccccatacctggcatataggaaggacatttcccctcctcccacttgctctgcttattatatgtaataggggtgtggaggaggcaagggagctgaattgggggcagataggggaacagtttggagatttatacaatctttgtgaatatcttcctttttttcttcgagttaggttagactaggacattgcctgcttccagcagcaccaccaggactgctgctggaaggacttcagagggtcaagaaaattctccaaagatttttgtgtctcaggcgatcccagcctcctctgtatttccagggacctgaggttacaggtggggattatcagaatatcagagagggtcctcgcccaaacaacaggatgccccaaactgaaggcttgtcatttatctctgaaagaggcaagtcaacaccttaatcctcatcatagcatagtcctcggtcctcagtggcaagggtgacttgaaagtggggcctttcatagctccagagccaaggaggccttgacaattaggcagagagaagacctggatgtccatcccatctgataccctgacttcccaagagaacaacccattcttctcagatttctcccaagtccctcattgctgggcctggaggctcgctttggctcctgtggtctctggaggatgcaggcatgaagcctgacctgacttgtactgaccctgtcccaggccttttgtgtctcgcctacctggctactcctcgtggccctacctatccaacagactgtgtgcaggtgggcaaggccaggctgtcttccaggagtcagtcccaacactcatcagcaaaaaggggtccgtgtctaggtgtctgggactggtttaagtaagaagagagtgccaagacccctctctctcttccagggagtgaactgatttctgacttgagttgtttaaattgggaagaggcctcatcagcaatcagagaggtctagatctctggaatctggccacggagtgattttcccatcagcctctgtctcggtgactgaggatctcggggcttcttcttttgcctctgacccaaggcccctcacacacttcttccagtgagccaggcagtgatgggcagaggagcggatctctccactccgtagagcatagatgacagggttgaccatggagttgatgaggcacagcatggagcagaaagcaaaggccttcttgacctggtcactgagcgtagtggccaggctgtgggccatgagggccagcactgggaaccaacagatgaggagcacagccaacactagccctagggtcttggccaacctcacatccagcctcattcgggccattcctggcacctgcctgtcctggtggccagacaagctggccacatgctgatgggccttccagagaacatgcccataggtgtagatgattccggaaaagaggaaggcgatgaacaggagccagctcagcaggtagtcattggggatcagtgggaaaagctcagagcagggcctgggacagcaagtccatcccatgaggggcaggtaggagactagtgctgagaggacccacatgatgcccagggtcaccagtgcccttccacgggtgagcagagctttgtaggaaggtggatagcgcaggcagaggtatcggtcaatggcggtcagcaggaggctacccacagaggctgtgaaggtcatagtcacgctgccaatcttcagcaggaagacagccttggaatccacaccatggaaaacatggaaattcacaaagctgcatgcaaagaccacactggccaggaagtcagccccagccaagctgccaatgaacaggtatgagggcttccggcggagttggtgggaggacaggatcagatagagcacagccacgttctccagggcacttagcaggcccagaagagtgcacaacacagcaacagctgtcttctggggaccactcaggatcatgtaatccttcatagggttggaatccaagccatccttggagccattggctatctctgtcacccagcattcctccatggggtgggcccttcagattccactgagcttgtctagaaggctttgggttgtgttgtgggtggctgggcactgggagctgccgggggctgaggagtcccagttgttttctgtcctctcccaggacctggccgtgggtgccactcagagcacctgttgagtgcc

SEQ ID NO: 11481 - RNA, 5815 nt, Homo sapiens
  source 1..5815: mol_type = other RNA
ctgaatagctgggactacaggtgcctgccaccatgccgggctaatttttgtatttttagcaaagatagggtttcactatgtcagccaggctggtcttgaactcccgaccttgtgatctgcttgccttggcctcccaaagttctgggattacaggcatgagccactatgcctcgcccagaaactgagtttctactctggcaagttaaacataaaaaattagtacatatcaggctgggtggctctaggccacatgcaagcaagctgcaaactgaattgcctctgcagctgcagaaggctaatttctacattgatatttggaaacactaacagctagaaaacaccactctactcatttttaaaaataagatcatattaaatgatgttacatgcatcatttatatattgctcacagtgccagcatcctcaaatatggttttaattttggtagatatcttgctagggggagcacatttccaagttatccagatatagggccctctttccttctctttctgtccacatgcaaccagatgctttgtggagttaaagttgacatttatttaaatgccacttggtgtctggtttttcacctttaatttagggttttctagctgggatgtaaaagaatcacttggagggatttttcaaaataccaatggccaggccactagccagtcaatcagaagcaaaatctccttggatgggacctggaaatctttagagttttccagcattttaatgaacatccctgattaagaaccaccgggtcttaagagtgtggcatatgtatttttcaagttcctagaggctctccaaaacaaaacaaaaaaaatctgctttattctctgcctggtgttgatgcatcagtctctttagccgttagtctgatcctggaaatttatggtcataatttgatgagcaatgttgggaatgacttcttctttttttttttttttttttgttttgagacagagtctcactctgttgaccaggctggagtgtagtggggcgatctccgctcactgcaacctccaccccaatactttcatttttaaatattatttatggcatccagatttgcataagatggactgggtcaatggccatgccctttataaatcaatattcttaagttctgcaaattcagtttcctaaagagccaaatcacatcctactcatcagcaaggcgggtagacatcattttcacaatcacttctaattttccaccattgtaaaaaaaaataaaatatgtaatcactttcttattgtaaaataaagaatttacttttccaggacctactgcctccctgtcccccccccccctttttttttttcaaacaatcttgaaccctttgtcacgagtcagttgccaagagaagcctatttgttggtttgagagcagttcatgcagacacagaccacttcctctgagaattcatttgcttcctcaggatggaatctggctgggcctctgaccttgctggtcacgtgggccggggcctccatcagtcataccctggactcctatctgtgtctaaacaccacgccccacccccaactgcacggcagccactcgcatagcactctgggagggctgtgggcatgagcagcgaggactccatcagcagctcccccacatgagccctgctgatgagggggcttgcgaagcagctttgatgtgctggtaaatccaggtgcaaaacagaactcaagttaaggcctccgcacagcactgcgttctaactgtgaaggattcttactctagtgtcctgtgtggaggtattggaattgtccattgctaagactcagaggagaaaagcacttagcatcgcaggacttggagcaccggtgctgaggcaacccttcattcattcgtcggatgtgtgttaaggcccagggcaggggtcacggattctcctctcacacagcacgtgggtggcaggaccaacaccgggtctgacctcccagccgggggcacaggctgctcaccccaggcctggaatctgtcagatgcccttcccgtgctgacttgacttagacaggcctcctgaccttcccacaaaggtcatgtgtgatttgcaggggttctggccgcttgaaaggttcctgagaaagcacatgcaatgaggacagagcttgcagagggaggacaggcatgcagaaggctctgtgtgcagccccagacctgggtaccttcatcaccgtcctcaccccacctccgggtgtgcacatagggagcaggtctcctgtgttatggcccaagcagggctgttaggacactgagaacattccctcctcccgcaggagagagaggtccaaggtgccctacatcgtgcgccagtgcgtggaggagatcgagcgccgaggcatggaggaggtgggcatctaccgcatgtctggggtggccgcagacatccaggcactgaaggcagccttcaacgtcagtgagtgtcggcctgcgcaggacgggatggaggtgtgggcagtggtgtccgcgatgagatctcagagtgctccacggcccaggcatgtcacatccttctctgtgtcttttcttcatttatcaggatcttcaaggaggccgctgcatttccgtgctctttccagataacaaggacgtgtcggtgatgatgagcgagatggacgtgaacgccatcgcaggcacgctgaagctgtatttccgtgagctgcccgagcccctcttcactgacgagttctaccccaacttcgcagagggcatcggtgagcactggaggccttggcctcatgggagacgtctcctccacgtgcactgctgccctcagaggctgtgaaaagtgaggtgtgggaacctgagctgtgcttcctctgccatggtcggaattttaacccaacctcaaaaagcaggggaccaaaactgagcctatcctggaaggccttgcccatccccagaggggtccccatccatatttctcaaggaggccaagtgggtgaaatggtcagcactgccgtgctgtggggtcctaaagtctgctgtcctccttcctgcagaccagggctaaacactggtgcccaggtgctcttgccatgggtcctggtccagccaagcatggtttcaaacatgacctgacccttagtcaacctggaggctgatgtctagagtgggcgctggagcgtgcagcacctgtagcctgtgcatcacccttagggcaggtctgcctcccgggcccatgcacagaggacctggtctcccagcctgcaggtgcccctgtggtgtccaggacaacgaggggttctctgcgtacttggtggggctgggaccctcccacttcccacctccttgtgtccctcactcccctgtttcattccatgctgagcctcccctgccttgggctccctggggagggggtggtggcaggagttgcccgagggcagctctgcccatgagcagctgctctagcggctcctcctgctgctgtttgccgggtgctgctgaccccaaggctggagtcagcttgcagcacagccagggtcgaggtcactccctccctgaggactctagcacggcacagcccctctgcctctctcctggtggtggcgttgaaacagcaccctctgcttcggtcctctaataagatgctggaatgtaatcctggacaatccgtgtcctggcagcatttggtcttcctctaagcgcctggctccgctgttctcaggagtgggttctgaagtctccgcctcctgcctcaacagcctgtgtggtggcaaagccggtgtggggctggggaacgcagcgttctccaggagggggacccggctctccttctgcaatgcaggcgaaggcctagatgccagtgtgacctcccacaaggcgtggcttccagactccccggccggaagtgatgcttttttgccgtgggccctgggtttgaagcagcctggctttctcttggtaagtggctggtgtcttagcagctgcaatctgagctcagccacctacacaccaccgtggccgacactttcattaagaagtttcctgagacgacttgcgtgcatgttgacttcatgatcagcgccgctgggaagaacccctgagccggtggggtggggctgtggccaccgctctggcacgagcccctcagtcttgggtggtttttgcctggtccaggatttggtgttgctgctgagttcagcctttccaccacctccgcatgggctgtgggtgttgtcagctgcctcccgccttggcttcagtagctcacccagcttacaggggagctgccctgggctggagatgggcacgcaccctgggtcctacttgaatgaatgcagcttgaggagacccggccatatacactgggccacgggttaccttcggcaatgcccacatcagctgtcagcctgagcctccccaggagagcaaggctcacatgacaaaggctgcccgtggccaatgaggtggctgagcccagccaggacctttctcggactcccgggatgtggctctgctcgtgagctgcctggtcagctctctcggggtgagaggggcttgtcacacgggcccctgcctgcagtgtgacccttctcagcttctctcagcagccctgcctgcggagtgtcaccgccaccatgatcatttccctgacactgcgagggtgtggggacgtcctgggtagagacagggcccatggcagcagcaggctcaggggcgccctgcactggtgggctggggacctggtggagaccacgccaagggctggacaaggggacgagcctccaccctggcctctccgcaggcctcagcagcccctcccacaggcagaagggttgacactgggttctgccctcactgcaagagctgcaagtgccatgtgctgttctgcccaatctggtgtctgcaggtgagggaagggctgccgctggcccgtttctgagtgttcagcacctaagggtgacagcactgtctgtccctaccctccaggtcctgtttgaaaatcaaacccatgctcacaggccaatttttttttcttttagagacagggtctcactttgtcacccaagctggagtgcagtggtgcgattatagctcaatgcagcctccaattcccggactcaagggaccttcctgcctcagcctgccaagtagcttggactatagctgtgtgttttattattattttgtagacatggggtctggctatgttgtccaggctattctcaaaattcccggcctcgagcaatcctcctgccttggcctctcaaaggttgggattacaggtgtgaggcaaggcacccagctcagccacagagccctgttgcatctctcttactaggagcaagagctgactgccccctcatccccattccagagtgttggggctgtgttgagccgaggccaggccactggcatgggcccagggagcgggatcattcactgctgccccaaatctgagatcattccaccttgacaagacttcctcatccaatccctttacttgacagctggggaaaccaatgcgcacagagcacccccagctcactcggggtctcagagctgatccatgagcagaggctgagatcctgggatcttgtcccccagcctccctgcaagcttactccctttctgctggaagagatggggccggacctcgaccagcagccctggcctggacgtgactgtgctcatgcaggtattgaggccgagatgccccagcatcatatgtttttctttttttttttctttcttttttgagattggctcactgcaacctctgcctcccgcttaaagtgattctcctgcctcagtcttccaagtagctgggcctacaggcttgta

SEQ ID NO: 11482 - RNA, 6337 nt, Homo sapiens
  source 1..6337: mol_type = other RNA
ctgaatagctgggactacaggtgcctgccaccatgccgggctaatttttgtatttttagcaaagatagggtttcactatgtcagccaggctggtcttgaactcccgaccttgtgatctgcttgccttggcctcccaaagttctgggattacaggcatgagccactatgcctcgcccagaaactgagtttctactctggcaagttaaacataaaaaattagtacatatcaggctgggtggctctaggccacatgcaagcaagctgcaaactgaattgcctctgcagctgcagaaggctaatttctacattgatatttggaaacactaacagctagaaaacaccactctactcatttttaaaaataagatcatattaaatgatgttacatgcatcatttatatattgctcacagtgccagcatcctcaaatatggttttaattttggtagatatcttgctagggggagcacatttccaagttatccagatatagggccctctttccttctctttctgtccacatgcaaccagatgctttgtggagttaaagttgacatttatttaaatgccacttggtgtctggtttttcacctttaatttagggttttctagctgggatgtaaaagaatcacttggagggatttttcaaaataccaatggccaggccactagccagtcaatcagaagcaaaatctccttggatgggacctggaaatctttagagttttccagcattttaatgaacatccctgattaagaaccaccgggtcttaagagtgtggcatatgtatttttcaagttcctagaggctctccaaaacaaaacaaaaaaaatctgctttattctctgcctggtgttgatgcatcagtctctttagccgttagtctgatcctggaaatttatggtcataatttgatgagcaatgttgggaatgacttcttctttttttttttttttttttgttttgagacagagtctcactctgttgaccaggctggagtgtagtggggcgatctccgctcactgcaacctccaccccaatactttcatttttaaatattatttatggcatccagatttgcataagatggactgggtcaatggccatgccctttataaatcaatattcttaagttctgcaaattcagtttcctaaagagccaaatcacatcctactcatcagcaaggcgggtagacatcattttcacaatcacttctaattttccaccattgtaaaaaaaaataaaatatgtaatcactttcttattgtaaaataaagaatttacttttccaggacctactgcctccctgtcccccccccccctttttttttttcaaacaatcttgaaccctttgtcacgagtcagttgccaagagaagcctatttgttggtttgagagcagttcatgcagacacagaccacttcctctgagaattcatttgcttcctcaggatggaatctggctgggcctctgaccttgctggtcacgtgggccggggcctccatcagtcataccctggactcctatctgtgtctaaacaccacgccccacccccaactgcacggcagccactcgcatagcactctgggagggctgtgggcatgagcagcgaggactccatcagcagctcccccacatgagccctgctgatgagggggcttgcgaagcagctttgatgtgctggtaaatccaggtgcaaaacagaactcaagttaaggcctccgcacagcactgcgttctaactgtgaaggattcttactctagtgtcctgtgtggaggtattggaattgtccattgctaagactcagaggagaaaagcacttagcatcgcaggacttggagcaccggtgctgaggcaacccttcattcattcgtcggatgtgtgttaaggcccagggcaggggtcacggattctcctctcacacagcacgtgggtggcaggaccaacaccgggtctgacctcccagccgggggcacaggctgctcaccccaggcctggaatctgtcagatgcccttcccgtgctgacttgacttagacaggcctcctgaccttcccacaaaggtcatgtgtgatttgcaggggttctggccgcttgaaaggttcctgagaaagcacatgcaatgaggacagagcttgcagagggaggacaggcatgcagaaggctctgtgtgcagccccagacctgggtaccttcatcaccgtcctcaccccacctccgggtgtgcacatagggagcaggtctcctgtgttatggcccaagcagggctgttaggacactgagaacattccctcctcccgcaggagagagaggtccaaggtgccctacatcgtgcgccagtgcgtggaggagatcgagcgccgaggcatggaggaggtgggcatctaccgcatgtctggggtggccgcagacatccaggcactgaaggcagccttcaacgtcagtgagtgtcggcctgcgcaggacgggatggaggtgtgggcagtggtgtccgcgatgagatctcagagtgctccacggcccaggcatgtcacatccttctctgtgtcttttcttcatttatcaggatcttcaaggaggccgctgcatttccgtgctctttccagataacaaggacgtgtcggtgatgatgagcgagatggacgtgaacgccatcgcaggcacgctgaagctgtatttccgtgagctgcccgagcccctcttcactgacgagttctaccccaacttcgcagagggcatcggtgagcactggaggccttggcctcatgggagacgtctcctccacgtgcactgctgccctcagaggctgtgaaaagtgaggtgtgggaacctgagctgtgcttcctctgccatggtcggaattttaacccaacctcaaaaagcaggggaccaaaactgagcctatcctggaaggccttgcccatccccagaggggtccccatccatatttctcaaggaggccaagtgggtgaaatggtcagcactgccgtgctgtggggtcctaaagtctgctgtcctccttcctgcagaccagggctaaacactggtgcccaggtgctcttgccatgggtcctggtccagccaagcatggtttcaaacatgacctgacccttagtcaacctggaggctgatgtctagagtgggcgctggagcgtgcagcacctgtagcctgtgcatcacccttagggcaggtctgcctcccgggcccatgcacagaggacctggtctcccagcctgcaggtgcccctgtggtgtccaggacaacgaggggttctctgcgtacttggtggggctgggaccctcccacttcccacctccttgtgtccctcactcccctgtttcattccatgctgagcctcccctgccttgggctccctggggagggggtggtggcaggagttgcccgagggcagctctgcccatgagcagctgctctagcggctcctcctgctgctgtttgccgggtgctgctgaccccaaggctggagtcagcttgcagcacagccagggtcgaggtcactccctccctgaggactctagcacggcacagcccctctgcctctctcctggtggtggcgttgaaacagcaccctctgcttcggtcctctaataagatgctggaatgtaatcctggacaatccgtgtcctggcagcatttggtcttcctctaagcgcctggctccgctgttctcaggagtgggttctgaagtctccgcctcctgcctcaacagcctgtgtggtggcaaagccggtgtggggctggggaacgcagcgttctccaggagggggacccggctctccttctgcaatgcaggcgaaggcctagatgccagtgtgacctcccacaaggcgtggcttccagactccccggccggaagtgatgcttttttgccgtgggccctgggtttgaagcagcctggctttctcttggtaagtggctggtgtcttagcagctgcaatctgagctcagccacctacacaccaccgtggccgacactttcattaagaagtttcctgagacgacttgcgtgcatgttgacttcatgatcagcgccgctgggaagaacccctgagccggtggggtggggctgtggccaccgctctggcacgagcccctcagtcttgggtggtttttgcctggtccaggatttggtgttgctgctgagttcagcctttccaccacctccgcatgggctgtgggtgttgtcagctgcctcccgccttggcttcagtagctcacccagcttacaggggagctgccctgggctggagatgggcacgcaccctgggtcctatgtgtttcaggaactgaggttcagctggcagtgggatgaggctggcccccttctccgctttcgttccgggaggcctcccgtagagcggtaggggctcgagatggcatttcgtttggggcacgagctggtccgggaggtctgggatctctggttctgacctctgggcacctgctgcagctgtggctgaggcccagaaatgtgaagggcctccatccactccagtagtgaccccaacgtggggttcaatgtggaggggggaggggctgctgcggcagctgcaggagcagaagtgccacaccttgttcttctcatgcccacatccatgcttgcagctgggaagggggcaggaatcagcgaggtgacctgggctgagtcctgggaatgggaagaggtggcaggaaggggatctgaggaggagaacagggggcctggtggtttgtgcttcttcccagacatgggagctgtagaggggacacctgcagcagatgctaagggggccagtaggcccaggcagtcttgggacttgtgtgtctcctgctgtacatccatactgggtgctttagaaatggcaggcagaccagaagtccctgttgcaagtgaggacaaagtgtgggaaggtcgtgagggtctgcagtccgagatggccttgtcctcaacctgcagtgcactgttgatgcgctggaatgccgcctccttctcccggtccaggtcttcaacagtgacccggtaccccagctctaagggaggtggcagcatcaaaggctcccctcgcctgcgtggcagcaggggaaacttgtgtgtactgggcctagaggcctcggatgtggaggagtcattcctgagggcgagtgtctgccctggtgctatatctgctgccttttcacactgggtgtgacctgaagagacagcctgaggcctgtcctcactcactgtctttgaggaactgagggtcagctggcagtgggatgaggctggccccctcctccgctttagccccggcaagcctcccgtggagctgtaggagctggagatggcatttcggttggtgcaggagctcgtccaggaggtctgggatgtctggttatatctgatttctgacctctgggcatggaggtctgtctgcagaggcccgggcccgggcacaaagggagagaggcctctattgtcccgcaggggccgaaatgcagacggtgcatccccggtgacctcggggacccttctctgatcaccaggattctcttggactctagggtccttgtcctgctcaggcatccctgccccgctctccttgagggccctcaacactatcttccctggacacaagtctggggacagccgggtgttgtggaccccaaaggggtgactcccggctcctgggccccacagagagtccatgttctcagtgcagtggctgagctggaggacgccctggaactcggagcacacagcactggcttgctgtggtacctgtgcaatcaaattgaaggcaggatcccaggaaggaaggcagggcttgcaggatcacggaaaaccttcttagagttgtcttgacaccactgatgtcaagtgtccgggtgcttgtaggatggcctgccactcagtccacgggcaggagcaacggggagatcccacaggcaaagtgaactgggggatgggctgaacgggctccaggcaactgagccctactggcaggtcctcggcctgggcccgaacaggaaggaggggcacagagtgcccaggtaaccgctcctgggagcagtggggaaccgtcggttgcttgaactctcgagagctgggctctgagcgtcctcgtccagccgccaactcggccaacggctaagccagcagtttcttctgttgccgggcaacgcgccttttaaacctgagggagcgggcgcgtgagcacatcacggcgcccgtgacagagcgagcttaacggattaataagcgcagccaggtacccgcgcgaggcgcttgctggcaatggcgggaggcggacgtggggggtcatgcaataggtactggaaggagagaggcgagc

SEQ ID NO: 11483 - RNA, 4017 nt, Homo sapiens
  source 1..4017: mol_type = other RNA
ctgaatagctgggactacaggtgcctgccaccatgcctggctagtttttttttgttttttttttttgtatttttagtagagacggggtttcaccgtgttagccaggatggtcttgatctccctacctcgtgatccgcccacctcggcctcccaaagtgctgggattacaggcgtgagccactgcgccccaccccattttggtgtgatctcagctcactgcaacctacccctcccaagttcaagtgattctcctacctcagcctcttgagtagctgggattacaggggtctgccaccacgcctggctgattttcctatttttagttgacactgcatttcaccaggttggccaggctggtcttgaactcctgacctcagctgatccacccgcctcgggctcccaaagtgttgggattacaggtgtgagccaccacaccaggcccatattttcttttagacatgcaggcaatgttgtggtttgttgttaagatgtcttaatattcctcttcccaggctctgaaacctagtgtgaaggtatatgctgctgaaccctcaaatgcagatgactgctaccagtccaagctgaaggggaaactgatgcccaatctttatcctccagaaaccatagcagatggtgtcaaatccagcattggcttgaacacctggcctattatcagggaccttgtggatgatatcttcactgtcacagaggatgaaattaaggtgaggctccagcaagaaaagaaatagcaaagcatggtgtaacttcttaggcagaagaaacttcccttaggagtagcaagtgacccacgggaacctgactaggtaacttcatgacatgggagggtaccctagatgtattaatgacaaccctcttgacagaagcagagtcagaattaaagaaaagctttgggaagcgtgtgtacacagtgataagaaaattcaaactggacacgtattctcatctgaactttataggtaaaccaactagactcccctttcactaattcctactcccttccatatcaacagtgtgcaacccagctggtgtgggagaggatgaaactactcattgaacctacagctggtgttggagtggctgctgtgctgtctcaacattttcaaactgtttccccagaagtaaagaacatttgtattgtgctcagtggtggaaatgtagacttaacctcctccataacttgggtgaagcaggctgaaaggccagcttcttatcagtctgtttctgtttaatttacagaaaaggaaatggtgggaattcagtgtctttagatactgaagacattttgtttcctagtattgtcaactcttagttatcagattcttaatggagagtggctatttcattaagatttaatagttttttttggactaagtagtggaaaaacttttatacttaactgagacattttgtcaaggctaaaaaaaagtcttgcaaaatggggcagtggactgacaggctgacatagaaaataaactttgcccaatcacaacttgtgcctcccatccctggagtactgactggcaccggtaagacagaatctctttgaatccattactccatgcccccttgaggcactgttgaagaaatctcacttttcagccagggtactggttctggtacatatggatcataagtccatttggggaagactcgtttatacaggttcatcagtactgtgtcttgagattttagcttcccatcaaagctgcatttcatgtggccatgggtacctaaaggttccttgatatgtcctctccggccccacttcgttctcagttccactggtttaaaccacagcacatcctctctgttgaagaacatgtaacgtactactgccatcttagtaaaaattttgaaaggatgaccactcagaacaactctcttgatgaccattctgtctggatctactgacataagatggcctgtagcaatgaggctgtgcattccattgcttttttgcttgaaaagcagcacagatgcaggaggaaaagtgattggcgcatagactgtcgccaccagggccatgtcagcagtcaggaatctctgcaatttatgtttgtccgctgcagtgtgctgagagaataaaggtgaggctcggaagcgcctgaatccacagtgaaatatgagctcttccttggctttcacaggttcagtgttgccagggtcacgcctcaccaccatattcaatactgacatcttctgttcatgaggtagtaaagaaaatgcaatcaagggtgttccttgcctgaagcactcgaccactgagacggggacttcagagacatgaagtgtgacataccagccaacctcagctccttcaacctctttttcttcaacctctttaaagatgcttttcctagtgttagtaaagttctgaaactgaaatattcgagcataatcttgaggaaggttttccttaggatcccatggagatgtccggaagctcttaaggcctctgtatttctgaaatcgaattcgagcagccacatcacggggcgtgtccacttcatctggaaacatctcttccagtctttcttgtttatatttctccaacatttttgcctcagcttcttcatctactttcttatcatacagatcatcatgcacagactccccaatagtcatagtttcatattcttcctcttcttcactactctcatcctgagattcctcctccataaaatcctcatgttccatatcatcatattcatattcatctccttccccaccactttggctgccaccatccaaaatccattcagcttggtaactggatgttcctttggggaccttctttaccaccttagaactttccttcaagaaatcctttgcctcgctcagctcctcctcagtgggccaggtttgctctccctccattggatctgggataacctctgcttgcaaggattcctgtctaccagggtctgccttcattaggactttaagaccttcttccatatcatctacagcatccgtagcacaaatctccattgccatgtctgggtccttttggggtttaattcctctaggatttaaagggaaagggtctccgggggcatctatctgtttcatctggaaatcaccatatccaacgatatgcagcaacctattgacattcagagtctgccctcgaacatagcctgaaattttcaaggtgcccaccaagttattctcttcactaggaacaaaatcaacagcatgggcaaataggtaggcccgccgatctcgaaaagcaagatgctgttgcttctggttagccaactgcctaagcagcatccctgcctcctgttgagtgtctaacaagaggagtttgtcatgcggaaagcgcttctccactgctttacttagcttcttcctggtatctatttgtttcttcagtgggaggccagaaatcccctggacagctagtgtataggtcggaaggccctgagcaaagaggcaggaaagacagtaatcaccggtgctgtcccagccttctagtggatcaaggaggaacaggatggtatcagctactttagccatgtctaacacaacgtgcagatcccctggccttgctgaggtgaaaaaccaccgatgtttcaagcgggggcacagcagcataaagttctgggtgtttcccaattcattcaagtgtactgttccagtgtccctatcttgaagcagctgcatggcctctggcagggaaattctgctgtgcaggggcaccaccagtacctgatgaggagggccatccttgccacccagctgtctcttctctgccagaaccgcctccttcttctgctttcggagctggctggcgcgatgcctctggtcgactctgctgagttcttttctcaccttcttgcttagggttttcagtgccagacggcccttgccgtcccgctgtgcagatccccgaccccgatgccgtccgcctttatgagctttattctgctgcttgagcgggccggggcggtgggccgccatgccgcagcgcgcgtgtacggagtcagcact

SEQ ID NO: 11484 - RNA, 2262 nt, Homo sapiens
  source 1..2262: mol_type = other RNA
ctgaatagctgggactacaggtgcctgccaccatgcttggctaatttttgtatttttagtagaattggggtttctccatgttggccaggctggtctagaactcctgacctcaagtgatctgcccacctcagcctctcaaagtgctgggattacaggtgtaagccaccacggcaagccctgtttttgtaaataaaggtttgttagagcatagaacacctgtttacttattgtttctggctgcttccacatagagttaaatagctgcaacagagaccatgtggctttgaaagcctgaaatgtttactctctggcccttcactgaaaaagttttctaaggtttgctgtagagctctcttccttagggtggatagtggaattgctactgatcatagatgatatctccaaatgagagaatgtggagacagaaggatgagagtgaggaggaggaaaatgtttgcatttcaggcttggaagagaaggaagctagggagggaggggagaggagagagaacaaaagtactgagtaatatcgtggaatctgagggaggccagagatgtttttgttgttttggtggtaacatgtaacatacaatttatcattactgacatttagtacatttacgaggtcgtaccttctttaccactctagttccagaacactttttgatcactccggaaggagagcccatacccattcatcagtcactccccatcccctcctttcccagcccctggcagcacaaatttacattctgtcttgtatgtttttccctttgccttagatctgggaaaggttttttttcgtcatggtggggaaatgggcttctgtgcagtcaggggagaagccgatggaggaaaggagtagtgtggttatggaagaggctgaaggggagaaggtcgcgggcatctggaggcctgagatgtgcatgagcatccagtcctgcaccggcgctggtgctgcagtggtgccgtctctgtcactgcagtgctgttctctgagagctgttccgcagcgtgattttgggtgctgttcctcattatgaagcctctcagtcatcttcttcagtctgcactgtacctttcatagatttctgattcaattagctgcagattggtttttgtggcttcctacctgaattctggccttggaattaagataaatctgtttaaaaaacgggctcagctcaaggcagatcacttaaggtgggacggagagggtttggagtgtatattgaagaaaaggagagtgcttataaaggtgggggaggaaaaggaggacgtgaaggcccagaagtgctgagaagcacagaagggtggtgttggtgttggcttttcagtcttcattttcctctgtgagtggatccttttagatcagtggtgggatgtcataaacgtttaatcctgagtgacacagaaggtgacacaggcttgcactttatatccaagaggaaccaagcacactcagataggtgcctgccattcttgtttctctaggaaaagttcctaaaggtgctaagaggggtacattttgtctaggttcagcactgggagggaggtgtaagaagctgcttgccttctttttaccttgtacttcactgcgtagacccagcacaggcttgggccacgtgccgagaaagggccgcacagccacaggttggctctcattgagcatggttatgtgttaactacccatatttcctggaaatgccacagaactgaagttggaagcaggtaggagagcctatgtctggacagcaaggggagtcctgggcagctgcacttacatggaccttggggagctggccccgttgttgccttgctgtcatggccactgagattcagctgctattgtgacccaggggacctctgtgtggcacagccttctgttctggaatcccagggaaacagctctggcctgcccgctccttcctatagttccagccacaattggcacctcactccctgcatccagtgcaatctcaggtgtctcctgctgtgcttgccttttccacagtcactctctaggaactactgaaattctcactagaatcagctgtttctctagatatggagcttgttccaaaagaatactttgcttttttgttgatgttctgacctttgatttcagtcctctccaaagataagaaacttgccatttgtagttgaagcatccataaagcatggttctgatgttggtggtgtaatagaattacttgggcaggttgaataactcttggctcttctatgcagttcagtgggctt

SEQ ID NO: 11485 - RNA, 2305 nt, Homo sapiens
  source 1..2305: mol_type = other RNA
ctgaatagctgggactacaggtgcctgccaccatgtccgactaatttttttgtatttttagtagagatggggtttcaccgtgttagacaggatggtctcgaactcctgaccttgtgatccgcccgcctcggcctcccaaagtgctgggattacaggtgtgagccaccgcgcccggcctggcagaaccttcttaacaagagggtccctccagcacatctttccgagagctaagttggtggggaaaacagactttgcactcatttggccgactgcctgagcagggtctgggaaaaatgcctttaaccccacctctgattccttgctcctatgctagaagactagcacatctatccctactgaacaaggagcttgtctggggttagggcactctcatcaaaaggcatctttgatgtttttgagctggcgcacagccagatctacagggaggctaaacttgaggctgctgaggcgactgagcaggttgagggcactctcaaagcctgtgtgtgccatgtagctccagggctggtagtgaggctcgatgagtgacccggacttgcagatgaggttcacccaggacaccagacgctgctcattcagtgccatgcacaccaaggccttcaattctgagtctgcactgcgcttaaaagggtcatgctctgtcagcaccatgtggatggctgtcagtaggctctgtttgggggtgacaacagtgcctcccgtaacaggaagggcgaaggactgggagagcttccgggctggggattccacataagcacggccgttcttagcatggtagtactttacaaagagctcccacgggtgcatggcctctggggccgaggagaaggctggcagcaaacaagcaataggagccataacaaggctcatccctggggaggaggcatacagtccatgggccagcaggtccctcacagccaccgttagctccttccgcacagccatagtcagctcatccttgcctcccagagagaggtcctggaggttggcagaggtgatgacatggtcatgtggctgctgcctcaaggctagctgcttcactctgtccactgacacctccagcctcttcagcaagggagagtagtctctgtcagcctggaccctctgccacagggttggagggatctggcctgtggcacaaccaaactggctaacagcaaagatctggagcacggccagcgctcgccgcatcaggtgcagccccgtctcccggactttcttcacatcctctgcctttgctgttttgctgtttcctggaggcgttctgctgctgcctgttctgctgcagccatttcctgtcttcccaccggccttgcactcacagtgtccaccacctgtctgcaaggggcttcccacttcatcttggatgaagttgataaacatctcaaggtctcggatctgagttttcagttgctcaaccaactgttctttgactcgggctgggttgacgatctgagccactgctgcatctacacgctgacgaagctcttcagtggacagggaactgatgtcctcattcagattcatgtccagtttctttattaactcatctatgatcacccgctgtctttccaacaccacggactgtggcagcgagtcataactgccctcttgataggcaaacgtttccaggtcatctagctgggtcttgagctgcagtatcagttctttctgcttctccctttgggtttccagacgctcttgcttttcctgctcactcaagccctggtcctcgccccgcaaccatggccggtcccctggcagcccatcgccctcatcgctggcggggtcgccgggcccttcgtaacctaggacgtgagggcagccgcggaaggcgaagtcttcgagctcccgcagaaggcgctgctgctccgccggcgccccgcgcaccacctggcgcaggcggaactgcacctgcgcgaagtgcgaggacagcgccagcagcgccgagtccagccgccgccgctctgcccgcagccgccgcagcgtccggcccggcgaatccggcggggagcccggggccgcgccaggctcctcggccgtcgcctcttctaaaaacgcggttgccccaggccgggcctccgccaccgcccccactggggcccagcgcaccgcctcgcacggtggcagcggctcctcttcctcctcctcttcgtctttcgcctttggcccaacagccgccaccaccgttaccggctctgcagccgcttcgacagccgccatcttcccggaaacaccaccgcacgtcagccgcgcccccctgctgccatggcaacggcgcggt

SEQ ID NO: 11486 - RNA, 2299 nt, Homo sapiens
  source 1..2299: mol_type = other RNA
ctgaatagctgggactacaggtgcctgccaccatgtccgactaatttttttgtatttttagtagagatggggtttcaccgtgttagacaggatggtctcgaactcctgaccttgtgatccgcccgcctcggcctcccaaagtgctgggattacaggtgtgagccaccgcgcccggcctggcagaaccttcttaacaagagggtccctccagcacatctttccgagagctaagttggtggggaaaacagactttgcactcatttggccgactgcctgagcagggtctgggaaaaatgcctttaaccccacctctgattccttgctcctatgctagaagactagcacatctatccctactgaacaaggagcttgtctggggttagggcactctcatcaaaaggcatctttgatgtttttgagctggcgcacagccagatctacagggaggctaaacttgaggctgctgaggcgactgagcaggttgagggcactctcaaagcctgtgtgtgccatgtagctccagggctggtagtgaggctcgatgagtgacccggacttgcagatgaggttcacccaggacaccagacgctgctcattcagtgccatgcacaccaaggccttcaattctgagtctgcactgcgcttaaaagggtcatgctctgtcagcaccatgtggatggctgtcagtaggctctgtttgggggtgacaacagtgcctcccgtaacaggaagggcgaaggactgggagagcttccgggctggggattccacataagcacggccgttcttagcatggtagtactttacaaagagctcccacgggtgcatggcctctggggccgaggagaaggctggcagcaaacaagcaataggagccataacaaggctcatccctggggaggaggcatacagtccatgggccagcaggtccctcacagccaccgttagctccttccgcacagccatagtcagctcatccttgcctcccagagagaggtcctggaggttggcagaggtgatgacatggtcatgtggctgctgcctcaaggctagctgcttcactctgtccactgacacctccagcctcttcagcaagggagagtagtctctgtcagcctggaccctctgccacagggttggagggatctggcctgtggcacaaccaaactggctaacagcaaagatctggagcacggccagcgctcgccgcatcaggtgcagccccgtctcccggactttcttcacatcctctgcctttgctgttttgctgtttcctggaggcgttctgctgctgcctgttctgctgcagccatttcctgtcttcccaccggccttgcactcacagtgtccaccacctgtctgcaaggggcttcccacttcatcttggatgaagttgataaacatctcaaggtctcggatctgagttttcagttgctcaaccaactgttctttgactcgggctgggttgacgatctgagccactgctgcatctacacgctgacgaagctcttcagtggacagggaactgatgtcctcattcagattcatgtccagtttctttattaactcatctatgatcacccgctgtctttccaacaccacggactgtggcagcgagtcataactgccctcttgataggcaaacgtttccaggtcatctagctgggtcttgagctgcagtatcagttctttctgcttctccctttgggtttccagacgctcttgcttttcctgctcactctggtcctcgccccgcaaccatggccggtcccctggcagcccatcgccctcatcgctggcggggtcgccgggcccttcgtaacctaggacgtgagggcagccgcggaaggcgaagtcttcgagctcccgcagaaggcgctgctgctccgccggcgccccgcgcaccacctggcgcaggcggaactgcacctgcgcgaagtgcgaggacagcgccagcagcgccgagtccagccgccgccgctctgcccgcagccgccgcagcgtccggcccggcgaatccggcggggagcccggggccgcgccaggctcctcggccgtcgcctcttctaaaaacgcggttgccccaggccgggcctccgccaccgcccccactggggcccagcgcaccgcctcgcacggtggcagcggctcctcttcctcctcctcttcgtctttcgcctttggcccaacagccgccaccaccgttaccggctctgcagccgcttcgacagccgccatcttcccggaaacaccaccgcacgtcagccgcgcccccctgctgccatggcaacggcgcggt

SEQ ID NO: 11487 - RNA, 2253 nt, Homo sapiens
  source 1..2253: mol_type = other RNA
ctgaatagctgggactacaggtgcctgccaccatgtccgactaatttttttgtatttttagtagagatggggtttcaccgtgttagacaggatggtctcgaactcctgaccttgtgatccgcccgcctcggcctcccaaagtgctgggattacaggtgtgagccaccgcgcccggcctggcagaaccttcttaacaagagggtccctccagcacatctttccgagagctaagttggtggggaaaacagactttgcactcatttggccgactgcctgagcagggtctgggaaaaatgcctttaaccccacctctgattccttgctcctatgctagaagactagcacatctatccctactgaacaaggagcttgtctggggttagggcactctcatcaaaaggcatctttgatgtttttgagctggcgcacagccagatctacagggaggctaaacttgaggctgctgaggcgactgagcaggttgagggcactctcaaagcctgtgtgtgccatgtagctccagggctggtagtgaggctcgatgagtgacccggacttgcagatgaggttcacccaggacaccagacgctgctcattcagtgccatgcacaccaaggccttcaattctgagtctgcactgcgcttaaaagggtcatgctctgtcagcaccatgtggatggctgtcagtaggctctgtttgggggtgacaacagtgcctcccgtaacaggaagggcgaaggactgggagagcttccgggctggggattccacataagcacggccgttcttagcatggtagtactttacaaagagctcccacgggtgcatggcctctggggccgaggagaaggctggcagcaaacaagcaataggagccataacaaggctcatccctggggaggaggcatacagtccatgggccagcaggtccctcacagccaccgttagctccttccgcacagccatagtcagctcatccttgcctcccagagagaggtcctggaggttggcagaggtgatgacatggtcatgtggctgctgcctcaaggctagctgcttcactctgtccactgacacctccagcctcttcagcaagggagagtagtctctgtcagcctggaccctctgccacagggttggagggatctggcctgtggcacaaccaaactggctaacagcaaagatctggagcacggccagcgctcgccgcatcaggtgcagccccgtctcccggactttcttcacatcctctgcctttgttttgctgtttcctggaggcgttctgctgctgcctgttctgctgcagccatttcctgtcttcccaccggccttgcactcacagtgtccaccacctgtctgcaaggggcttcccacttcatcttggatgaagttgataaacatctcaaggtctcggatctgagttttcagttgctcaaccaactgttctttgactcgggctgggttgacgatctgagccactgctgcatctacacgctgacgaagctcttcagtggacagggaactgatgtcctcattcagattcatgtccagtttctttattaactcatctatgatcacccgctgtctttccaacaccacggactgtggcagcgagtcataactgccctcttgataggcaaacgtttccaggtcatctagctgggtcttgagctgcagtatcagttctttctgcttctccctttgggtttccagacgctcttgcttttcctgctcactcaagccctggtcctcgccccgcaaccatggccggtcccctggcagcccatcgccctcatcgctggcggggtcgccgggcccttcgtaacctaggacgtgagggcagccgcggaaggcgaagtcttcgagctcccgcagaaggcgctgctgctccgccggcgccccgcgcaccacctggcgcaggcggaactgcacctgcgcgaagtgcgaggacagcgccagcagcgccgagtccagccgccgccgctctgcccgcagccgccgcagcgtccggcccggcgaatccggcggggagcccggggccgcgccaggctcctcggccgtcgcctcttctaaaaacgcggttgccccaggccgggcctccgccaccgcccccactggggcccagcgcaccgcctcgcacggtggcagcggctcctcttcctcctcctcttcgtctttcgcctttggcccaacagccgccaccaccgttaccggctctgcagccgcttcgacagccgccatcttcccggaaac

SEQ ID NO: 11488 - RNA, 2247 nt, Homo sapiens
  source 1..2247: mol_type = other RNA
ctgaatagctgggactacaggtgcctgccaccatgtccgactaatttttttgtatttttagtagagatggggtttcaccgtgttagacaggatggtctcgaactcctgaccttgtgatccgcccgcctcggcctcccaaagtgctgggattacaggtgtgagccaccgcgcccggcctggcagaaccttcttaacaagagggtccctccagcacatctttccgagagctaagttggtggggaaaacagactttgcactcatttggccgactgcctgagcagggtctgggaaaaatgcctttaaccccacctctgattccttgctcctatgctagaagactagcacatctatccctactgaacaaggagcttgtctggggttagggcactctcatcaaaaggcatctttgatgtttttgagctggcgcacagccagatctacagggaggctaaacttgaggctgctgaggcgactgagcaggttgagggcactctcaaagcctgtgtgtgccatgtagctccagggctggtagtgaggctcgatgagtgacccggacttgcagatgaggttcacccaggacaccagacgctgctcattcagtgccatgcacaccaaggccttcaattctgagtctgcactgcgcttaaaagggtcatgctctgtcagcaccatgtggatggctgtcagtaggctctgtttgggggtgacaacagtgcctcccgtaacaggaagggcgaaggactgggagagcttccgggctggggattccacataagcacggccgttcttagcatggtagtactttacaaagagctcccacgggtgcatggcctctggggccgaggagaaggctggcagcaaacaagcaataggagccataacaaggctcatccctggggaggaggcatacagtccatgggccagcaggtccctcacagccaccgttagctccttccgcacagccatagtcagctcatccttgcctcccagagagaggtcctggaggttggcagaggtgatgacatggtcatgtggctgctgcctcaaggctagctgcttcactctgtccactgacacctccagcctcttcagcaagggagagtagtctctgtcagcctggaccctctgccacagggttggagggatctggcctgtggcacaaccaaactggctaacagcaaagatctggagcacggccagcgctcgccgcatcaggtgcagccccgtctcccggactttcttcacatcctctgcctttgttttgctgtttcctggaggcgttctgctgctgcctgttctgctgcagccatttcctgtcttcccaccggccttgcactcacagtgtccaccacctgtctgcaaggggcttcccacttcatcttggatgaagttgataaacatctcaaggtctcggatctgagttttcagttgctcaaccaactgttctttgactcgggctgggttgacgatctgagccactgctgcatctacacgctgacgaagctcttcagtggacagggaactgatgtcctcattcagattcatgtccagtttctttattaactcatctatgatcacccgctgtctttccaacaccacggactgtggcagcgagtcataactgccctcttgataggcaaacgtttccaggtcatctagctgggtcttgagctgcagtatcagttctttctgcttctccctttgggtttccagacgctcttgcttttcctgctcactctggtcctcgccccgcaaccatggccggtcccctggcagcccatcgccctcatcgctggcggggtcgccgggcccttcgtaacctaggacgtgagggcagccgcggaaggcgaagtcttcgagctcccgcagaaggcgctgctgctccgccggcgccccgcgcaccacctggcgcaggcggaactgcacctgcgcgaagtgcgaggacagcgccagcagcgccgagtccagccgccgccgctctgcccgcagccgccgcagcgtccggcccggcgaatccggcggggagcccggggccgcgccaggctcctcggccgtcgcctcttctaaaaacgcggttgccccaggccgggcctccgccaccgcccccactggggcccagcgcaccgcctcgcacggtggcagcggctcctcttcctcctcctcttcgtctttcgcctttggcccaacagccgccaccaccgttaccggctctgcagccgcttcgacagccgccatcttcccggaaac

SEQ ID NO: 11489 - RNA, 2943 nt, Homo sapiens
  source 1..2943: mol_type = other RNA
ctgaatagctgggactacaggtgcctgccaccattcccagttaatttttgtatttttagtagagatgacatttcactatgttggccaggctggttttgaactcctgacctcgtgatccacctgcctcagcttcccaaagtgctgggattacaggcatgagccaccacgcctggcccaaatcctatttttcaatatttatttcctaattatgtcctactaggttaggttttattttcatttgttacatatttattgggttatttcctttatgctaggaactttattagtataaggatacagataaggtccattctctgttctcaagaatctgagtctacaggcagaagacaaaatgcagtacagaattatggaaatgtgaatggaaactgcattcagagaggggtattgcttgggaaaagccacattggcgtgccacagatgtatgccagcctggcaggcccatagtgtgattacttgagtttcaatatctgattcttttataggcttgaaattggtttatcaggtctggaagtgactggactctggagtactgagttacccaccacaaactgctaataaaatgctgtgtaaaagccattaatactaatgtattatttatgagaaacacaattatggggaagctaggatagttgagtttgctggtcattatcttccttgtattgaccaaattacaatgaaggctaaatccaaattataatcagaagattgcttggtaaatacagaacagaaacaatagaaatgtgtgtggtgcttttaatggctagtatttcaagcctgatgcagccctttccacttgagtcacattgtcttacattctttgacttggctagtgctaaaaatacattgccattttactttctccattttttttttttttttttttttgagacgacgtctggattgcaattggtgtgaggttggctcactacaacctctgcctcccgggttcaagcgattctcctgccccagcctcctgagtagctgggactacaggtgcacgccaccacgcccagctaatttttgtatttttagtagagacggggtttcaccatgttggccaggatggtctccatctcttgacctcgtgatccacctgcctcggcctcccaaagtgctgggattacaggcgtgagccaccacgcccagcccatcctttctcctcttaaattttctttgctgaccagtatctcttgatgtggaacgttctttcattagtggtaatactgtcaatcaggtctttggaagatattttgggttttgtttgctgaaccattatgcttattttacaaattaacttttctgaactttattgtggtagaatttacataacaatttaccattttgaccatttttaagttcaaaggaactaagtacattcacattgctatgcaactatgactaccatctagctccagaaccttttcatcttctcaaactgaaattctgtacccattaaacaataagctcccagccgggcacagtggctcgcgcctgtaatcccagcactttgggaggctgaggtgggcggattacctggagtcaggagttcgagaccagcctggccaacatgatggccatctctactaagaatacaaaaattagctggttgtggtgatgaatgcctgtaatcccagctacgtgggaggctgaggcatgagaatcacttgaacctgggaggcagacgttgcagtgagctgggattgcaccactgcactccagcctaggcaacagaaggagactcccgtctcaaaaaaaaaaaaacaaaacaaaaacaagaaccaataagctcccattccttctgccttccagcccttggcaaccaccattccactttaaatttgattattctaggagttcataaaagtggggtaacacagtatttgtcattttgtgactgacttatttcacctatcataaagtcttcaagattcatccaagatgtaatatatatcagaagtttcctcctttttaaggctgagtaatattccattgtgtgtatatgtcacatttcttttaaccattcatcccttgatggacacttggattgcttccaccttctggctattgtgaatgctgctgctgtgaacatagatgtacaaattatctgtccaagttcctgcttttacttcttttgggtatatacccggaagtggaattgctggatataattttaatttttgaggaatctccatactcagatgatcttatttccttatttttcaagtgtgtgggtctatgtgtggttttggcagggaagcgagtctctgttattcccacatactccccatgactgttaagtgctgtgttagaagcatatggtttgatgagaattctaggagagacaaatgtttcaaaggatctctgtattttcaccggcaataactaataaatcatctggcttcgctgttccccaccatgtagttgtggcattttgggaattagtacactcaggagagaagctgtgtttaggatgaagtgagttggatcatacttcgtatagaaacttgccagaaaatatagaattattggagaaattgtgaaaaacttccgtgaagatgtaaactgtactccatagtccagttgttcccaatgagttaggagccttgctttaccctggtcaggagtttcgaaaggtgttcctttcactgcatgcaaaaatacgtacatccccagattatgtataatatttgttaaagtccaagcaacaggaacactgaagaagggaatgctgagtaagacaatatgaagcaagccaactcccaatgcatatgtcagccacataccccggctgttcatgacacgggtatttggattcacttcactgtgggcaactccaacgttcatgtttgctccgccgccccactccgggccgccggctcgcagcaggaccagcccggctgctacggccgcggatacacgccc

SEQ ID NO: 11490 - RNA, 2837 nt, Homo sapiens
  source 1..2837: mol_type = other RNA
ctgaatagctgggactacaggtgcctgccaccattcccagttaatttttgtatttttagtagagatgacatttcactatgttggccaggctggttttgaactcctgacctcgtgatccacctgcctcagcttcccaaagtgctgggattacaggcatgagccaccacgcctggcccaaatcctatttttcaatatttatttcctaattatgtcctactaggttaggttttattttcatttgttacatatttattgggttatttcctttatgctaggaactttattagtataaggatacagataaggtccattctctgttctcaagaatctgagtctacaggcagaagacaaaatgcagtacagaattatggaaatgtgaatggaaactgcattcagagaggggtattgcttgggaaaagccacattggcgtgccacagatgtatgccagcctggcaggcccatagtgtgattacttgagtttcaatatctgattcttttataggcttgaaattggtttatcaggtctggaagtgactggactctggagtactgagttacccaccacaaactgctaataaaatgctgtgtaaaagccattaatactaatgtattatttatgagaaacacaattatggggaagctaggatagttgagtttgctggtcattatcttccttgtattgaccaaattacaatgaaggctaaatccaaattataatcagaagattgcttggtaaatacagaacagaaacaatagaaatgtgtgtggtgcttttaatggctagtatttcaagcctgatgcagccctttccacttgagtcacattgtcttacattctttgacttggctagtgctaaaaatacattgccattttactttctccattttttttttttttttttttttgagacgacgtctggattgcaattggtgtgaggttggctcactacaacctctgcctcccgggttcaagcgattctcctgccccagcctcctgagtagctgggactacaggtgcacgccaccacgcccagctaatttttgtatttttagtagagacggggtttcaccatgttggccaggatggtctccatctcttgacctcgtgatccacctgcctcggcctcccaaagtgctgggattacaggcgtgagccaccacgcccagcccatcctttctcctcttaaattttctttgctgaccagtatctcttgatgtggaacgttctttcattagtggtaatactgtcaatcaggtctttggaagatattttgggttttgtttgctgaaccattatgcttattttacaaattaacttttctgaactttattgtggtagaatttacataacaatttaccattttgaccatttttaagttcaaaggaactaagtacattcacattgctatgcaactatgactaccatctagctccagaaccttttcatcttctcaaactgaaattctgtacccattaaacaataagctcccagccgggcacagtggctcgcgcctgtaatcccagcactttgggaggctgaggtgggcggattacctggagtcaggagttcgagaccagcctggccaacatgatggccatctctactaagaatacaaaaattagctggttgtggtgatgaatgcctgtaatcccagctacgtgggaggctgaggcatgagaatcacttgaacctgggaggcagacgttgcagtgagctgggattgcaccactgcactccagcctaggcaacagaaggagactcccgtctcaaaaaaaaaaaaacaaaacaaaaacaagaaccaataagctcccattccttctgccttccagcccttggcaaccaccattccactttaaatttgattattctaggagttcataaaagtggggtaacacagtatttgtcattttgtgactgacttatttcacctatcataaagtcttcaagattcatccaagatgtaatatatatcagaagtttcctcctttttaaggctgagtaatattccattgtgtgtatatgtcacatttcttttaaccattcatcccttgatggacacttggattgcttccaccttctggctattgtgaatgctgctgctgtgaacatagatgtacaaattatctgtccaagttcctgcttttacttcttttgggtatatacccggaagtggaattgctggatataattttaatttttgaggaatctccatactcagatgatcttatttccttatttttcaagtgtgtgggtctatgtgtggttttggcagggaagcgagtctctgttattcccacatactccccatgactgttaagtgctgtgttagaagcatatggtttgatgagaattctaggagagacaaatgtttcaaaggatctctgtattttcaccggcaataactaataaatcatctggcttcgctgttccccagaattattggagaaattgtgaaaaacttccgtgaagatgtaaactgtactccatagtccagttgttcccaatgagttaggagccttgctttaccctggtcaggagtttcgaaaggtgttcctttcactgcatgcaaaaatacgtacatccccagattatgtataatatttgttaaagtccaagcaacaggaacactgaagaagggaatgctgagtaagacaatatgaagcaagccaactcccaatgcatatgtcagccacataccccggctgttcatgacacgggtatttggattcacttcactgtgggcaactccaacgttcatgtttgctccgccgccccactccgggccgccggctcgcagcaggaccagcccggctgctacggccgcggatacacgccc

SEQ ID NO: 11491 - RNA, 2881 nt, Homo sapiens
  source 1..2881: mol_type = other RNA
ctgaatagctgggactacaggtgcctgccaccattcccagttaatttttgtatttttagtagagatgacatttcactatgttggccaggctggttttgaactcctgacctcgtgatccacctgcctcagcttcccaaagtgctgggattacaggcatgagccaccacgcctggcccaaatcctatttttcaatatttatttcctaattatgtcctactaggttaggttttattttcatttgttacatatttattgggttatttcctttatgctaggaactttattagtataaggatacagataaggtccattctctgttctcaagaatctgagtctacaggcagaagacaaaatgcagtacagaattatggaaatgtgaatggaaactgcattcagagaggggtattgcttgggaaaagccacattggcgtgccacagatgtatgccagcctggcaggcccatagtgtgattacttgagtttcaatatctgattcttttataggcttgaaattggtttatcaggtctggaagtgactggactctggagtactgagttacccaccacaaactgctaataaaatgctgtgtaaaagccattaatactaatgtattatttatgagaaacacaattatggggaagctaggatagttgagtttgctggtcattatcttccttgtattgaccaaattacaatgaaggctaaatccaaattataatcagaagattgcttggtaaatacagaacagaaacaatagaaatgtgtgtggtgcttttaatggctagtatttcaagcctgatgcagccctttccacttgagtcacattgtcttacattctttgacttggctagtgctaaaaatacattgccattttactttctccattttttttttttttttttttttgagacgacgtctggattgcaattggtgtgaggttggctcactacaacctctgcctcccgggttcaagcgattctcctgccccagcctcctgagtagctgggactacaggtgcacgccaccacgcccagctaatttttgtatttttagtagagacggggtttcaccatgttggccaggatggtctccatctcttgacctcgtgatccacctgcctcggcctcccaaagtgctgggattacaggcgtgagccaccacgcccagcccatcctttctcctcttaaattttctttgctgaccagtatctcttgatgtggaacgttctttcattagtggtaatactgtcaatcaggtctttggaagatattttgggttttgtttgctgaaccattatgcttattttacaaattaacttttctgaactttattgtggtagaatttacataacaatttaccattttgaccatttttaagttcaaaggaactaagtacattcacattgctatgcaactatgactaccatctagctccagaaccttttcatcttctcaaactgaaattctgtacccattaaacaataagctcccagccgggcacagtggctcgcgcctgtaatcccagcactttgggaggctgaggtgggcggattacctggagtcaggagttcgagaccagcctggccaacatgatggccatctctactaagaatacaaaaattagctggttgtggtgatgaatgcctgtaatcccagctacgtgggaggctgaggcatgagaatcacttgaacctgggaggcagacgttgcagtgagctgggattgcaccactgcactccagcctaggcaacagaaggagactcccgtctcaaaaaaaaaaaaacaaaacaaaaacaagaaccaataagctcccattccttctgccttccagcccttggcaaccaccattccactttaaatttgattattctaggagttcataaaagtggggtaacacagtatttgtcattttgtgactgacttatttcacctatcataaagtcttcaagattcatccaagatgtaatatatatcagaagtttcctcctttttaaggctgagtaatattccattgtgtgtatatgtcacatttcttttaaccattcatcccttgatggacacttggattgcttccaccttctggctattgtgaatgctgctgctgtgaacatagatgtacaaattatctgtccaagttcctgcttttacttcttttgggtatatacccggaagtggaattgctggatataattttaatttttgaggaatctccatactcagatgatcttatttccttatttttcaagtgtgtgggtctatgtgtggttttggcagggaagcgagtctctgttattcccacatactccccatgactgttaagtgctgtgttagaagcatatggtttgatgagaattctaggagagacaaatgtttcaaaggatctctgtattttcaccggcaataactaataaatcatctggcttcgctgttccccagaattattggagaaattgtgaaaaacttccgtgaagatgtaaactgtactccatagtccagttgttcccaatgagttaggagccttgctttaccctggtcaggagtttcgaaaggtgttcctttcactgcatgcaaaaatacgtacatccccagattatgtataatatttgttaaagtccaagcaacaggaacactgaagaagggaatgctgagtaagacaatatgaagcaagccaactcccaatgcatatgtcagccacataccccggctgttcatgacacgggtatttggattcacttcactgtgggcaactccaacgttcatgtttgctcgtgaagaggctgttggctctgccctcgccggtgcctccgaagacggcgacccgcagcggcccctcaggggagtcccccctgctagaccgacagcccgagcgctctgggccagag

SEQ ID NO: 11492 - RNA, 3032 nt, Homo sapiens
  source 1..3032: mol_type = other RNA
ctgaatagctgggactacaggtgcctgccaccattcccagttaatttttgtatttttagtagagatgacatttcactatgttggccaggctggttttgaactcctgacctcgtgatccacctgcctcagcttcccaaagtgctgggattacaggcatgagccaccacgcctggcccaaatcctatttttcaatatttatttcctaattatgtcctactaggttaggttttattttcatttgttacatatttattgggttatttcctttatgctaggaactttattagtataaggatacagataaggtccattctctgttctcaagaatctgagtctacaggcagaagacaaaatgcagtacagaattatggaaatgtgaatggaaactgcattcagagaggggtattgcttgggaaaagccacattggcgtgccacagatgtatgccagcctggcaggcccatagtgtgattacttgagtttcaatatctgattcttttataggcttgaaattggtttatcaggtctggaagtgactggactctggagtactgagttacccaccacaaactgctaataaaatgctgtgtaaaagccattaatactaatgtattatttatgagaaacacaattatggggaagctaggatagttgagtttgctggtcattatcttccttgtattgaccaaattacaatgaaggctaaatccaaattataatcagaagattgcttggtaaatacagaacagaaacaatagaaatgtgtgtggtgcttttaatggctagtatttcaagcctgatgcagccctttccacttgagtcacattgtcttacattctttgacttggctagtgctaaaaatacattgccattttactttctccattttttttttttttttttttttgagacgacgtctggattgcaattggtgtgaggttggctcactacaacctctgcctcccgggttcaagcgattctcctgccccagcctcctgagtagctgggactacaggtgcacgccaccacgcccagctaatttttgtatttttagtagagacggggtttcaccatgttggccaggatggtctccatctcttgacctcgtgatccacctgcctcggcctcccaaagtgctgggattacaggcgtgagccaccacgcccagcccatcctttctcctcttaaattttctttgctgaccagtatctcttgatgtggaacgttctttcattagtggtaatactgtcaatcaggtctttggaagatattttgggttttgtttgctgaaccattatgcttattttacaaattaacttttctgaactttattgtggtagaatttacataacaatttaccattttgaccatttttaagttcaaaggaactaagtacattcacattgctatgcaactatgactaccatctagctccagaaccttttcatcttctcaaactgaaattctgtacccattaaacaataagctcccagccgggcacagtggctcgcgcctgtaatcccagcactttgggaggctgaggtgggcggattacctggagtcaggagttcgagaccagcctggccaacatgatggccatctctactaagaatacaaaaattagctggttgtggtgatgaatgcctgtaatcccagctacgtgggaggctgaggcatgagaatcacttgaacctgggaggcagacgttgcagtgagctgggattgcaccactgcactccagcctaggcaacagaaggagactcccgtctcaaaaaaaaaaaaacaaaacaaaaacaagaaccaataagctcccattccttctgccttccagcccttggcaaccaccattccactttaaatttgattattctaggagttcataaaagtggggtaacacagtatttgtcattttgtgactgacttatttcacctatcataaagtcttcaagattcatccaagatgtaatatatatcagaagtttcctcctttttaaggctgagtaatattccattgtgtgtatatgtcacatttcttttaaccattcatcccttgatggacacttggattgcttccaccttctggctattgtgaatgctgctgctgtgaacatagatgtacaaattatctgtccaagttcctgcttttacttcttttgggtatatacccggaagtggaattgctggatataattttaatttttgaggaatctccatactcagatgatcttatttccttatttttcaagtgtgtgggtctatgtgtggttttggcagggaagcgagtctctgttattcccacatactccccatgactgttaagtgctgtgttagaagcatatggtttgatgagaattctaggagagacaaatgtttcaaaggatctctgtattttcaccggcaataactaataaatcatctggcttcgctgttcccccactccttccttataagaaattcagtagctgtaaaattttttttcagtttcaaaacatttcaatacttattaattccaaagatccgaacaccatgtagttgtggcattttgggaattagtacactcaggagagaagctgtgtttaggatgaagtgagttggatcatacttcgtatagaaacttgccagaaaatatagaattattggagaaattgtgaaaaacttccgtgaagatgtaaactgtactccatagtccagttgttcccaatgagttaggagccttgctttaccctggtcaggagtttcgaaaggtgttcctttcactgcatgcaaaaatacgtacatccccagattatgtataatatttgttaaagtccaagcaacaggaacactgaagaagggaatgctgagtaagacaatatgaagcaagccaactcccaatgcatatgtcagccacataccccggctgttcatgacacgggtatttggattcacttcactgtgggcaactccaacgttcatgtttgctccgccgccccactccgggccgccggctcgcagcaggaccagcccggctgctacggccgcggatacacgccc

SEQ ID NO: 11493 - RNA, 2966 nt, Homo sapiens
  source 1..2966: mol_type = other RNA
ctgaatagctgggactacaggtgcctgccaccattcccagttaatttttgtatttttagtagagatgacatttcactatgttggccaggctggttttgaactcctgacctcgtgatccacctgcctcagcttcccaaagtgctgggattacaggcatgagccaccacgcctggcccaaatcctatttttcaatatttatttcctaattatgtcctactaggttaggttttattttcatttgttacatatttattgggttatttcctttatgctaggaactttattagtataaggatacagataaggtccattctctgttctcaagaatctgagtctacaggcagaagacaaaatgcagtacagaattatggaaatgtgaatggaaactgcattcagagaggggtattgcttgggaaaagccacattggcgtgccacagatgtatgccagcctggcaggcccatagtgtgattacttgagtttcaatatctgattcttttataggcttgaaattggtttatcaggtctggaagtgactggactctggagtactgagttacccaccacaaactgctaataaaatgctgtgtaaaagccattaatactaatgtattatttatgagaaacacaattatggggaagctaggatagttgagtttgctggtcattatcttccttgtattgaccaaattacaatgaaggctaaatccaaattataatcagaagattgcttggtaaatacagaacagaaacaatagaaatgtgtgtggtgcttttaatggctagtatttcaagcctgatgcagccctttccacttgagtcacattgtcttacattctttgacttggctagtgctaaaaatacattgccattttactttctccattttttttttttttttttttttgagacgacgtctggattgcaattggtgtgaggttggctcactacaacctctgcctcccgggttcaagcgattctcctgccccagcctcctgagtagctgggactacaggtgcacgccaccacgcccagctaatttttgtatttttagtagagacggggtttcaccatgttggccaggatggtctccatctcttgacctcgtgatccacctgcctcggcctcccaaagtgctgggattacaggcgtgagccaccacgcccagcccatcctttctcctcttaaattttctttgctgaccagtatctcttgatgtggaacgttctttcattagtggtaatactgtcaatcaggtctttggaagatattttgggttttgtttgctgaaccattatgcttattttacaaattaacttttctgaactttattgtggtagaatttacataacaatttaccattttgaccatttttaagttcaaaggaactaagtacattcacattgctatgcaactatgactaccatctagctccagaaccttttcatcttctcaaactgaaattctgtacccattaaacaataagctcccagccgggcacagtggctcgcgcctgtaatcccagcactttgggaggctgaggtgggcggattacctggagtcaggagttcgagaccagcctggccaacatgatggccatctctactaagaatacaaaaattagctggttgtggtgatgaatgcctgtaatcccagctacgtgggaggctgaggcatgagaatcacttgaacctgggaggcagacgttgcagtgagctgggattgcaccactgcactccagcctaggcaacagaaggagactcccgtctcaaaaaaaaaaaaacaaaacaaaaacaagaaccaataagctcccattccttctgccttccagcccttggcaaccaccattccactttaaatttgattattctaggagttcataaaagtggggtaacacagtatttgtcattttgtgactgacttatttcacctatcataaagtcttcaagattcatccaagatgtaatatatatcagaagtttcctcctttttaaggctgagtaatattccattgtgtgtatatgtcacatttcttttaaccattcatcccttgatggacacttggattgcttccaccttctggctattgtgaatgctgctgctgtgaacatagatgtacaaattatctgtccaagttcctgcttttacttcttttgggtatatacccggaagtggaattgctggatataattttaatttttgaggaatctccatactcagatgatcttatttccttatttttcaagtgtgtgggtctatgtgtggttttggcagggaagcgagtctctgttattcccacatactccccatgactgttaagtgctgtgttagaagcatatggtttgatgagaattctaggagagacaaatgtttcaaaggatctctgtattttcaccggcaataactaataaatcatctggcttcgctgttccccttattaattccaaagatccgaacaccatgtagttgtggcattttgggaattagtacactcaggagagaagctgtgtttaggatgaagtgagttggatcatacttcgtatagaaacttgccagaaaatatagaattattggagaaattgtgaaaaacttccgtgaagatgtaaactgtactccatagtccagttgttcccaatgagttaggagccttgctttaccctggtcaggagtttcgaaaggtgttcctttcactgcatgcaaaaatacgtacatccccagattatgtataatatttgttaaagtccaagcaacaggaacactgaagaagggaatgctgagtaagacaatatgaagcaagccaactcccaatgcatatgtcagccacataccccggctgttcatgacacgggtatttggattcacttcactgtgggcaactccaacgttcatgtttgctccgccgccccactccgggccgccggctcgcagcaggaccagcccggctgctacggccgcggatacacgccc

SEQ ID NO: 11494 - RNA, 3076 nt, Homo sapiens
  source 1..3076: mol_type = other RNA
ctgaatagctgggactacaggtgcctgccaccattcccagttaatttttgtatttttagtagagatgacatttcactatgttggccaggctggttttgaactcctgacctcgtgatccacctgcctcagcttcccaaagtgctgggattacaggcatgagccaccacgcctggcccaaatcctatttttcaatatttatttcctaattatgtcctactaggttaggttttattttcatttgttacatatttattgggttatttcctttatgctaggaactttattagtataaggatacagataaggtccattctctgttctcaagaatctgagtctacaggcagaagacaaaatgcagtacagaattatggaaatgtgaatggaaactgcattcagagaggggtattgcttgggaaaagccacattggcgtgccacagatgtatgccagcctggcaggcccatagtgtgattacttgagtttcaatatctgattcttttataggcttgaaattggtttatcaggtctggaagtgactggactctggagtactgagttacccaccacaaactgctaataaaatgctgtgtaaaagccattaatactaatgtattatttatgagaaacacaattatggggaagctaggatagttgagtttgctggtcattatcttccttgtattgaccaaattacaatgaaggctaaatccaaattataatcagaagattgcttggtaaatacagaacagaaacaatagaaatgtgtgtggtgcttttaatggctagtatttcaagcctgatgcagccctttccacttgagtcacattgtcttacattctttgacttggctagtgctaaaaatacattgccattttactttctccattttttttttttttttttttttgagacgacgtctggattgcaattggtgtgaggttggctcactacaacctctgcctcccgggttcaagcgattctcctgccccagcctcctgagtagctgggactacaggtgcacgccaccacgcccagctaatttttgtatttttagtagagacggggtttcaccatgttggccaggatggtctccatctcttgacctcgtgatccacctgcctcggcctcccaaagtgctgggattacaggcgtgagccaccacgcccagcccatcctttctcctcttaaattttctttgctgaccagtatctcttgatgtggaacgttctttcattagtggtaatactgtcaatcaggtctttggaagatattttgggttttgtttgctgaaccattatgcttattttacaaattaacttttctgaactttattgtggtagaatttacataacaatttaccattttgaccatttttaagttcaaaggaactaagtacattcacattgctatgcaactatgactaccatctagctccagaaccttttcatcttctcaaactgaaattctgtacccattaaacaataagctcccagccgggcacagtggctcgcgcctgtaatcccagcactttgggaggctgaggtgggcggattacctggagtcaggagttcgagaccagcctggccaacatgatggccatctctactaagaatacaaaaattagctggttgtggtgatgaatgcctgtaatcccagctacgtgggaggctgaggcatgagaatcacttgaacctgggaggcagacgttgcagtgagctgggattgcaccactgcactccagcctaggcaacagaaggagactcccgtctcaaaaaaaaaaaaacaaaacaaaaacaagaaccaataagctcccattccttctgccttccagcccttggcaaccaccattccactttaaatttgattattctaggagttcataaaagtggggtaacacagtatttgtcattttgtgactgacttatttcacctatcataaagtcttcaagattcatccaagatgtaatatatatcagaagtttcctcctttttaaggctgagtaatattccattgtgtgtatatgtcacatttcttttaaccattcatcccttgatggacacttggattgcttccaccttctggctattgtgaatgctgctgctgtgaacatagatgtacaaattatctgtccaagttcctgcttttacttcttttgggtatatacccggaagtggaattgctggatataattttaatttttgaggaatctccatactcagatgatcttatttccttatttttcaagtgtgtgggtctatgtgtggttttggcagggaagcgagtctctgttattcccacatactccccatgactgttaagtgctgtgttagaagcatatggtttgatgagaattctaggagagacaaatgtttcaaaggatctctgtattttcaccggcaataactaataaatcatctggcttcgctgttccccttattaattccaaagatccgaacaccatgtagttgtggcattttgggaattagtacactcaggagagaagctgtgtttaggatgaagtgagttggatcatacttcgtatagaaacttgccagaaaatatagaattattggagaaattgtgaaaaacttccgtgaagatgtaaactgtactccatagtccagttgttcccaatgagttaggagccttgctttaccctggtcaggagtttcgaaaggtgttcctttcactgcatgcaaaaatacgtacatccccagattatgtataatatttgttaaagtccaagcaacaggaacactgaagaagggaatgctgagtaagacaatatgaagcaagccaactcccaatgcatatgtcagccacataccccggctgttcatgacacgggtatttggattcacttcactgtgggcaactccaacgttcatgtttgctcgagccagtgtgtcaagtagtcagactcttatatttgacttaatgtatccataaagaatggtcagagttcagatcacttctttctgaatactcaatgtggaaggtacatgccgccgccccactccgggccgccggctcgcagcaggaccagcccggctgctacggccgcggatacacgccc

SEQ ID NO: 11495 - RNA, 6265 nt, Homo sapiens
  source 1..6265: mol_type = other RNA
ctgaatagctgggactacaggtgcctgccacctcgcccagctaattttttgtatttttagtagagacggggtttcaccgtgttagccaggatggtctcgatctcctgacctcgtgatccgcccaccttagcctcccaaagtgctgggattacaggcgtgagccaccacgcccggcctcatttacaaattttctaaataaacgtcctgagaaaagagacaaaaggaagggaaatcttttcctttattctcaaaggaggaattatgcctctcatttatttgcttgtttgagacagggtctagctctgtcacccaggctggagtgcagtggtgagatcagggctcacttcagcctcaaaatccctgcttcaactgatcctcccacttcagtgcccagagtagctgggaccacagcagtgcaccaccacacctggctgactttttttacttttagcagagaagaggtcccctatgtcgcccaggctggtcttgaatccctaggctcacgtcacccacctgcctgggcctctaaaaccgctgggattacaggcctgagccactgcgtctggtctcatcgtaaatttgatgtttcttcttgttttaacagaatttgtattgctgtgatagaggttcttttcaaactgatgtcttatccttctgagtgcctcaaactagagcctgttcagacgttataacaagtttatactggtttattttggtacaaaaagtgtgaaatttatgcacaaatttttcataatatgtatttttccatgaacttcttgaagacccttatactagcaaactgtattcaagaggatataaaaagggattgtaaacatccaagtgctacctattcatgggatgcaaggatggttcaacatactcaaatcaatgggatacacacttgcacagaatgacagataaaaaacacattatctcaatagatagagaaaaagcatttcacagaactcaatattcattcttcgtaaaaatcctaaacaatataggtagagttttacctcaaaaatataaaaatcatccatgaaatgaccacagctgaaataaccaatgaaggaaaatggaatggttttcctgtaggatatcacatgatgcaagaatgctctcacccctgatattcaataaatactggctgtcctaggcagagcaattaaatagcaaaagaaataaaactcatccaaatcagaaagacagaagtaaaattacatttgttggggccgggctcatggctcacacccataatcccagcaatttgcaagtccgaagtgggcggataatgaggttaggcgatctaacatattctttcaagttctcttcaaggtactcaccatgttggcccaccatctgggccaacatggtgaaaccccgtctttactaaaataaaaaaaataaataaattagctaggtgtggtgacatgcgcctgtagtcccagctactcaggaggctgagacagaattgcttggacgtgggagacagaggttgcagtgagcaaagatcattccacggcactctagcctggcgacagagagagacattgtctcaaaaaaaaaaattatttccttgtagatgatacgacattctatatagaaaatcactggctgggtgcggtggctcacacctgtaatcccagaactttgggatgctgatgggggcggatcacctgaagtcaggagttcaagaaaaacctggtcaacatggtgaaaccccgtctctactaaaaatacaaaaaaattatacggacatggtggcaggcacctgtaatctcagttagtaggcaggagaatcacttaaacccgaaaggcagaggctgcagtgagccaagatcgtgccattgtactccagtccaagtgacaagagtgagactccttctcaaaaaaaaagaaaagagcctgggtaacagagtgagactgtctcaaaaaaaaaagaaagaaaatcacaaagaatcaaccaagattttactgatactaataaacccactcaatgtatttgcagaatacaaaatcagcacccaaaattagttgaatttccttacattaacaataaataatgtttaaagaaacttatgaacacacttcaatttgctatgaaacttaatacttacaaataaactgaattaaggaggtgagaagcttgtaccttgaaatctacattgatcaaaaaaactaaatagacatacaacccatattgatggattggaagtcttaatattgttgaatgattatacaaacaaatgtgatttagattcaacagatacccataaaaacccgtaacagtttttattaaagaaacaaaatacagggtgggaaaagtgactcatgtctgttggccagtctggtctcaaactcctgacctcaagtgatctattggtcttggcctcccaaagtgctgggattacaggcgtgagccaccccgcctggcccaatcttcttaacataaacactttaatgtcaattaatgcttgaactcaatgttaagtcaattcaaactcaagtcaatgctgaattgactctaatgccaattaatgcttgatggtttgctatactcattgcatttggaacaatcatctcaaaaatgaattttctgatgttccttaaggggtgatctcagactgaagaccttgccacactgatgacatttgtaagatttctgtccagtatggattctctgatgtctaattaggtgtgaacgtgaagtaaaggctttgctgcaatcatcatacttgtgaagtttgtctcctgtatgaagtctcctgttttgcataagatgaagctagactgaagaccttgccacaatcatgacatttgtaaggtttctctccagcatgagttcaccgatgaactgcaaggtatgaacaatgtctgaaaaatttgccacatttattacactttcaaaatctctcattatggattctccaatgatttgaaacggttgtagtgttactgaagactttgtgataatcattacattagtaaagtttccctataccatggattgcctgatggtgaataagtgttgactgcccactaaaggctttgccacactcagtacacttgtaaggtttctctccagtgtgacttctagtttgttgggccaggtgtgaatcacgcccaagattcttgtcacaaactcttacatttgtaagctttctctccagtatgaattctcctgtctttcaagacttgatttacaactgtaaactttgtcacattcttcatatttctaatgtttctttccagtatgaattctatgatgacgtgcaagttttgcttttcgattaaaaaccttgccacattcattacacttgtaaggtttctctccagtatgaattgtcttatgaattacaaggactgaattgtgacggaaggttttgccacactcattacacttgtaaggtttctctccagtatgaattctatgatgacatgcaaggtgtgcttgttgattaaaaaccttaccacatttattacacttgtaaggtttctctccagtatgaagtctatgatgacgtgaaaggtttgcttttctattaaaaaccttgccacattcactacacttgtaaggtttttctccagtatgaattgccttatgaatttcaagggctgaattgtgacggaaggtcttgccacactcattacacttgtaaggtttctctccactatgaattgccttatgaattacaagggctgaattgtgacggaagttcttgccacattcattacacttgtaaggtttctctccagtgtgaattctagtatgttgtgccaggtgtgaatcacgcccaaaagctttgtcacaaaccttacatttgtatggtttctctccagtatgaattctcctgtgtttttcaaggcttgatttgcgactgaaaactttgtcacattcttcacatttgtaaggtttctctccagtatgaagtctaagatggcatgtaagggatgacttctgactgaaggccttgccacactcattacacttgtaaggtttctctccagtatgaattgccttgtgaattataagggctgaatttcgaccgaaggtcttgccacactcattacacttgtaaggtttctctccagtatgaagtctacgatggcatgtaaggtatgacttccgactaaaggtcttgccacattcattacacctgtaaggtttctctccagtatgaattctcctatgtctttgaaggtttgatttgaaactgaaagcttcatcacattcttcacatttgtaaggtttctctccactatgagttcgccaatgaactgcaaggtatgaacgatgtctgaaaaatttgccacatctattacacttgtacgatctctcttcattatggattctccaatgatttgcaatggttgtagcattactaaagacttggtgacaatcattacatttgtaaagtttccctataccatggattgcttgatggtaaataagtgctgactgcccacgaaaggctttgccacactcattacactggtaaggtttctctccagtatgaagtctacaatggcgtgtaagggatgacttccgactaaaggtcttgccacattcattacacttgtaaagtttctctccagtatgaattatcctatgtctttcaaggtttgatttgaaactgaaagcttcatcacattcttcacatttgtaaggtttctctccagtatgaagtctacgatggtatacaagggatgatgtctgactgaaggtcttgccacaatcattacacttgtaaggtttctctccagtatgaattctcctatgtctttcaaggttcgatttgaaactgaaagcttcatcacattcttcacatttgtaaggtttctctccagtatgaagtctacgatggtatacaagggatgacatctgactgaaggtcttgccacaatcattacacttataaggtttctctccagtatgaagtctacgatggcgtgtaagggatgacttccgactaaaggtcctgctgcattcattacacttgtaaggtttctctccagtatgaattttcctatgtctttcaaggtttgatttgaaactgaaagctttgtcacattcttcacatttgtaaggtttctctccagtatgaagtctacgatggtacacaaggtatgacgtttgactgaaggtcttgccacattcattacacttgtaagatttctctccagtatgaattgccttatgaattacaagggctgaatttcgactgaaggtcttgccacactcactgcacttgtaatgtttctctccagtatgaagtctatgatggcatgtaagggttaactcctgactgaaggtcttgccacaatcattacacttgtaaggtttcttgccagtgtgacatctacgatgacatgcaagatatcgcttttgattaaagaccttgccacacacatcacatttatattgtttcgctcctaaatggattatctgatgtttccttaagactgagctataattaaaggctttgccactctcattacattggaaagatttttctctcatgtgtacttcctgcttttgtgtgagtaatgaagaattcaggaaattattcccatagttcttagaaatgtgggttttaggcctacaagaaattctttgggatgttgaaaccaacgaagcactgttgatagacttctcaacttgattaccaattttcccttcggtctgaaacatgtggagttcaggcagatgcgaatgaaagcttgatccaagctgatctttaataggcttgtttccagcatgcctttgatcatgtcggtttgtactacccgtcaactgtttgatttctgtcatgggtgcttcatggctatttctttcatcttctttccactgaaactcaaaatcatgaatatctttctccatttcctggaagcaaaaatctccaatgtgatgacgttcatgtctttgcaatgtccctgtgtggatcacttctgtattgccttgtgctgttgatgagaactccttcatcatgcatttggaagagatatccagggagaccaggttcctataattctccagcatcacgtccctgtatagagtcctctgagcagggtccaggcacttccactcttcctgagagaattctatggccacatccctgaatgtcaatagaccctgagaaagagccatccctgactcctttgctttcctcttcctcttccgggtttcttcctcacgtaccaagagtctttagaagtcaatccgctgcggtgggaccatcactccatgcgatccgcttccgggttt

SEQ ID NO: 11496 - RNA, 6359 nt, Homo sapiens
  source 1..6359: mol_type = other RNA
ctgaatagctgggactacaggtgcctgccacctcgcccagctaattttttgtatttttagtagagacggggtttcaccgtgttagccaggatggtctcgatctcctgacctcgtgatccgcccaccttagcctcccaaagtgctgggattacaggcgtgagccaccacgcccggcctcatttacaaattttctaaataaacgtcctgagaaaagagacaaaaggaagggaaatcttttcctttattctcaaaggaggaattatgcctctcatttatttgcttgtttgagacagggtctagctctgtcacccaggctggagtgcagtggtgagatcagggctcacttcagcctcaaaatccctgcttcaactgatcctcccacttcagtgcccagagtagctgggaccacagcagtgcaccaccacacctggctgactttttttacttttagcagagaagaggtcccctatgtcgcccaggctggtcttgaatccctaggctcacgtcacccacctgcctgggcctctaaaaccgctgggattacaggcctgagccactgcgtctggtctcatcgtaaatttgatgtttcttcttgttttaacagaatttgtattgctgtgatagaggttcttttcaaactgatgtcttatccttctgagtgcctcaaactagagcctgttcagacgttataacaagtttatactggtttattttggtacaaaaagtgtgaaatttatgcacaaatttttcataatatgtatttttccatgaacttcttgaagacccttatactagcaaactgtattcaagaggatataaaaagggattgtaaacatccaagtgctacctattcatgggatgcaaggatggttcaacatactcaaatcaatgggatacacacttgcacagaatgacagataaaaaacacattatctcaatagatagagaaaaagcatttcacagaactcaatattcattcttcgtaaaaatcctaaacaatataggtagagttttacctcaaaaatataaaaatcatccatgaaatgaccacagctgaaataaccaatgaaggaaaatggaatggttttcctgtaggatatcacatgatgcaagaatgctctcacccctgatattcaataaatactggctgtcctaggcagagcaattaaatagcaaaagaaataaaactcatccaaatcagaaagacagaagtaaaattacatttgttggggccgggctcatggctcacacccataatcccagcaatttgcaagtccgaagtgggcggataatgaggttaggcgatctaacatattctttcaagttctcttcaaggtactcaccatgttggcccaccatctgggccaacatggtgaaaccccgtctttactaaaataaaaaaaataaataaattagctaggtgtggtgacatgcgcctgtagtcccagctactcaggaggctgagacagaattgcttggacgtgggagacagaggttgcagtgagcaaagatcattccacggcactctagcctggcgacagagagagacattgtctcaaaaaaaaaaattatttccttgtagatgatacgacattctatatagaaaatcactggctgggtgcggtggctcacacctgtaatcccagaactttgggatgctgatgggggcggatcacctgaagtcaggagttcaagaaaaacctggtcaacatggtgaaaccccgtctctactaaaaatacaaaaaaattatacggacatggtggcaggcacctgtaatctcagttagtaggcaggagaatcacttaaacccgaaaggcagaggctgcagtgagccaagatcgtgccattgtactccagtccaagtgacaagagtgagactccttctcaaaaaaaaagaaaagagcctgggtaacagagtgagactgtctcaaaaaaaaaagaaagaaaatcacaaagaatcaaccaagattttactgatactaataaacccactcaatgtatttgcagaatacaaaatcagcacccaaaattagttgaatttccttacattaacaataaataatgtttaaagaaacttatgaacacacttcaatttgctatgaaacttaatacttacaaataaactgaattaaggaggtgagaagcttgtaccttgaaatctacattgatcaaaaaaactaaatagacatacaacccatattgatggattggaagtcttaatattgttgaatgattatacaaacaaatgtgatttagattcaacagatacccataaaaacccgtaacagtttttattaaagaaacaaaatacagggtgggaaaagtgactcatgtctgttggccagtctggtctcaaactcctgacctcaagtgatctattggtcttggcctcccaaagtgctgggattacaggcgtgagccaccccgcctggcccaatcttcttaacataaacactttaatgtcaattaatgcttgaactcaatgttaagtcaattcaaactcaagtcaatgctgaattgactctaatgccaattaatgcttgatggtttgctatactcattgcatttggaacaatcatctcaaaaatgaattttctgatgttccttaaggggtgatctcagactgaagaccttgccacactgatgacatttgtaagatttctgtccagtatggattctctgatgtctaattaggtgtgaacgtgaagtaaaggctttgctgcaatcatcatacttgtgaagtttgtctcctgtatgaagtctcctgttttgcataagatgaagctagactgaagaccttgccacaatcatgacatttgtaaggtttctctccagcatgagttcaccgatgaactgcaaggtatgaacaatgtctgaaaaatttgccacatttattacactttcaaaatctctcattatggattctccaatgatttgaaacggttgtagtgttactgaagactttgtgataatcattacattagtaaagtttccctataccatggattgcctgatggtgaataagtgttgactgcccactaaaggctttgccacactcagtacacttgtaaggtttctctccagtgtgacttctagtttgttgggccaggtgtgaatcacgcccaagattcttgtcacaaactcttacatttgtaagctttctctccagtatgaattctcctgtctttcaagacttgatttacaactgtaaactttgtcacattcttcatatttctaatgtttctttccagtatgaattctatgatgacgtgcaagttttgcttttcgattaaaaaccttgccacattcattacacttgtaaggtttctctccagtatgaattgtcttatgaattacaaggactgaattgtgacggaaggttttgccacactcattacacttgtaaggtttctctccagtatgaattctatgatgacatgcaaggtgtgcttgttgattaaaaaccttaccacatttattacacttgtaaggtttctctccagtatgaagtctatgatgacgtgaaaggtttgcttttctattaaaaaccttgccacattcactacacttgtaaggtttttctccagtatgaattgccttatgaatttcaagggctgaattgtgacggaaggtcttgccacactcattacacttgtaaggtttctctccactatgaattgccttatgaattacaagggctgaattgtgacggaagttcttgccacattcattacacttgtaaggtttctctccagtgtgaattctagtatgttgtgccaggtgtgaatcacgcccaaaagctttgtcacaaaccttacatttgtatggtttctctccagtatgaattctcctgtgtttttcaaggcttgatttgcgactgaaaactttgtcacattcttcacatttgtaaggtttctctccagtatgaagtctaagatggcatgtaagggatgacttctgactgaaggccttgccacactcattacacttgtaaggtttctctccagtatgaattgccttgtgaattataagggctgaatttcgaccgaaggtcttgccacactcattacacttgtaaggtttctctccagtatgaagtctacgatggcatgtaaggtatgacttccgactaaaggtcttgccacattcattacacctgtaaggtttctctccagtatgaattctcctatgtctttgaaggtttgatttgaaactgaaagcttcatcacattcttcacatttgtaaggtttctctccactatgagttcgccaatgaactgcaaggtatgaacgatgtctgaaaaatttgccacatctattacacttgtacgatctctcttcattatggattctccaatgatttgcaatggttgtagcattactaaagacttggtgacaatcattacatttgtaaagtttccctataccatggattgcttgatggtaaataagtgctgactgcccacgaaaggctttgccacactcattacactggtaaggtttctctccagtatgaagtctacaatggcgtgtaagggatgacttccgactaaaggtcttgccacattcattacacttgtaaagtttctctccagtatgaattatcctatgtctttcaaggtttgatttgaaactgaaagcttcatcacattcttcacatttgtaaggtttctctccagtatgaagtctacgatggtatacaagggatgatgtctgactgaaggtcttgccacaatcattacacttgtaaggtttctctccagtatgaattctcctatgtctttcaaggttcgatttgaaactgaaagcttcatcacattcttcacatttgtaaggtttctctccagtatgaagtctacgatggtatacaagggatgacatctgactgaaggtcttgccacaatcattacacttataaggtttctctccagtatgaagtctacgatggcgtgtaagggatgacttccgactaaaggtcctgctgcattcattacacttgtaaggtttctctccagtatgaattttcctatgtctttcaaggtttgatttgaaactgaaagctttgtcacattcttcacatttgtaaggtttctctccagtatgaagtctacgatggtacacaaggtatgacgtttgactgaaggtcttgccacattcattacacttgtaagatttctctccagtatgaattgccttatgaattacaagggctgaatttcgactgaaggtcttgccacactcactgcacttgtaatgtttctctccagtatgaagtctatgatggcatgtaagggttaactcctgactgaaggtcttgccacaatcattacacttgtaaggtttcttgccagtgtgacatctacgatgacatgcaagatatcgcttttgattaaagaccttgccacacacatcacatttatattgtttcgctcctaaatggattatctgatgtttccttaagactgagctataattaaaggctttgccactctcattacattggaaagatttttctctcatgtgtacttcctgcttttgtgtgagtaatgaagaattcaggaaattattcccatagttcttagaaatgtgggttttaggcctacaagaaattctttgggatgttgaaaccaacgaagcactgttgatagacttctcaacttgattaccaattttcccttcggtctgaaacatgtggagttcaggcagatgcgaatgaaagcttgatccaagctgatctttaataggcttgtttccagcatgcctttgatcatgtcggtttgtactacccgtcaactgtttgatttctgtcatgggtgcttcatggctatttctttcatcttctttccactgaaactcaaaatcatgaatatctttctccatttcctggaagcaaaaatctccaatgtgatgacgttcatgtctttgcaatgtccctgtgtggatcacttctgtattgccttgtgctgttgatgagaactccttcatcatgcatttggaagagatatccagggagaccaggttcctataattctccagcatcacgtccctgtatagagtcctctgagcagggtccaggcacttccactcttcctgagagaattctatggccacatccctgaatgtcaatagaccctgagaaagagccatccctgactcctttgctttcctcttcctcttccgggtttcttcctcacgtaccaagagtctttagaagtcaatcctgcagctgaggggccagcgagttccagcagagggacagcccacatgaacgccttgaggcaggagcaacctcggcccaggaacaggaaagacgccgctgcggtgggaccatcactccatgcgatccgcttccgggttt

SEQ ID NO: 11497 - RNA, 6367 nt, Homo sapiens
  source 1..6367: mol_type = other RNA
ctgaatagctgggactacaggtgcctgccacctcgcccagctaattttttgtatttttagtagagacggggtttcaccgtgttagccaggatggtctcgatctcctgacctcgtgatccgcccaccttagcctcccaaagtgctgggattacaggcgtgagccaccacgcccggcctcatttacaaattttctaaataaacgtcctgagaaaagagacaaaaggaagggaaatcttttcctttattctcaaaggaggaattatgcctctcatttatttgcttgtttgagacagggtctagctctgtcacccaggctggagtgcagtggtgagatcagggctcacttcagcctcaaaatccctgcttcaactgatcctcccacttcagtgcccagagtagctgggaccacagcagtgcaccaccacacctggctgactttttttacttttagcagagaagaggtcccctatgtcgcccaggctggtcttgaatccctaggctcacgtcacccacctgcctgggcctctaaaaccgctgggattacaggcctgagccactgcgtctggtctcatcgtaaatttgatgtttcttcttgttttaacagaatttgtattgctgtgatagaggttcttttcaaactgatgtcttatccttctgagtgcctcaaactagagcctgttcagacgttataacaagtttatactggtttattttggtacaaaaagtgtgaaatttatgcacaaatttttcataatatgtatttttccatgaacttcttgaagacccttatactagcaaactgtattcaagaggatataaaaagggattgtaaacatccaagtgctacctattcatgggatgcaaggatggttcaacatactcaaatcaatgggatacacacttgcacagaatgacagataaaaaacacattatctcaatagatagagaaaaagcatttcacagaactcaatattcattcttcgtaaaaatcctaaacaatataggtagagttttacctcaaaaatataaaaatcatccatgaaatgaccacagctgaaataaccaatgaaggaaaatggaatggttttcctgtaggatatcacatgatgcaagaatgctctcacccctgatattcaataaatactggctgtcctaggcagagcaattaaatagcaaaagaaataaaactcatccaaatcagaaagacagaagtaaaattacatttgttggggccgggctcatggctcacacccataatcccagcaatttgcaagtccgaagtgggcggataatgaggttaggcgatctaacatattctttcaagttctcttcaaggtactcaccatgttggcccaccatctgggccaacatggtgaaaccccgtctttactaaaataaaaaaaataaataaattagctaggtgtggtgacatgcgcctgtagtcccagctactcaggaggctgagacagaattgcttggacgtgggagacagaggttgcagtgagcaaagatcattccacggcactctagcctggcgacagagagagacattgtctcaaaaaaaaaaattatttccttgtagatgatacgacattctatatagaaaatcactggctgggtgcggtggctcacacctgtaatcccagaactttgggatgctgatgggggcggatcacctgaagtcaggagttcaagaaaaacctggtcaacatggtgaaaccccgtctctactaaaaatacaaaaaaattatacggacatggtggcaggcacctgtaatctcagttagtaggcaggagaatcacttaaacccgaaaggcagaggctgcagtgagccaagatcgtgccattgtactccagtccaagtgacaagagtgagactccttctcaaaaaaaaagaaaagagcctgggtaacagagtgagactgtctcaaaaaaaaaagaaagaaaatcacaaagaatcaaccaagattttactgatactaataaacccactcaatgtatttgcagaatacaaaatcagcacccaaaattagttgaatttccttacattaacaataaataatgtttaaagaaacttatgaacacacttcaatttgctatgaaacttaatacttacaaataaactgaattaaggaggtgagaagcttgtaccttgaaatctacattgatcaaaaaaactaaatagacatacaacccatattgatggattggaagtcttaatattgttgaatgattatacaaacaaatgtgatttagattcaacagatacccataaaaacccgtaacagtttttattaaagaaacaaaatacagggtgggaaaagtgactcatgtctgttggccagtctggtctcaaactcctgacctcaagtgatctattggtcttggcctcccaaagtgctgggattacaggcgtgagccaccccgcctggcccaatcttcttaacataaacactttaatgtcaattaatgcttgaactcaatgttaagtcaattcaaactcaagtcaatgctgaattgactctaatgccaattaatgcttgatggtttgctatactcattgcatttggaacaatcatctcaaaaatgaattttctgatgttccttaaggggtgatctcagactgaagaccttgccacactgatgacatttgtaagatttctgtccagtatggattctctgatgtctaattaggtgtgaacgtgaagtaaaggctttgctgcaatcatcatacttgtgaagtttgtctcctgtatgaagtctcctgttttgcataagatgaagctagactgaagaccttgccacaatcatgacatttgtaaggtttctctccagcatgagttcaccgatgaactgcaaggtatgaacaatgtctgaaaaatttgccacatttattacactttcaaaatctctcattatggattctccaatgatttgaaacggttgtagtgttactgaagactttgtgataatcattacattagtaaagtttccctataccatggattgcctgatggtgaataagtgttgactgcccactaaaggctttgccacactcagtacacttgtaaggtttctctccagtgtgacttctagtttgttgggccaggtgtgaatcacgcccaagattcttgtcacaaactcttacatttgtaagctttctctccagtatgaattctcctgtctttcaagacttgatttacaactgtaaactttgtcacattcttcatatttctaatgtttctttccagtatgaattctatgatgacgtgcaagttttgcttttcgattaaaaaccttgccacattcattacacttgtaaggtttctctccagtatgaattgtcttatgaattacaaggactgaattgtgacggaaggttttgccacactcattacacttgtaaggtttctctccagtatgaattctatgatgacatgcaaggtgtgcttgttgattaaaaaccttaccacatttattacacttgtaaggtttctctccagtatgaagtctatgatgacgtgaaaggtttgcttttctattaaaaaccttgccacattcactacacttgtaaggtttttctccagtatgaattgccttatgaatttcaagggctgaattgtgacggaaggtcttgccacactcattacacttgtaaggtttctctccactatgaattgccttatgaattacaagggctgaattgtgacggaagttcttgccacattcattacacttgtaaggtttctctccagtgtgaattctagtatgttgtgccaggtgtgaatcacgcccaaaagctttgtcacaaaccttacatttgtatggtttctctccagtatgaattctcctgtgtttttcaaggcttgatttgcgactgaaaactttgtcacattcttcacatttgtaaggtttctctccagtatgaagtctaagatggcatgtaagggatgacttctgactgaaggccttgccacactcattacacttgtaaggtttctctccagtatgaattgccttgtgaattataagggctgaatttcgaccgaaggtcttgccacactcattacacttgtaaggtttctctccagtatgaagtctacgatggcatgtaaggtatgacttccgactaaaggtcttgccacattcattacacctgtaaggtttctctccagtatgaattctcctatgtctttgaaggtttgatttgaaactgaaagcttcatcacattcttcacatttgtaaggtttctctccactatgagttcgccaatgaactgcaaggtatgaacgatgtctgaaaaatttgccacatctattacacttgtacgatctctcttcattatggattctccaatgatttgcaatggttgtagcattactaaagacttggtgacaatcattacatttgtaaagtttccctataccatggattgcttgatggtaaataagtgctgactgcccacgaaaggctttgccacactcattacactggtaaggtttctctccagtatgaagtctacaatggcgtgtaagggatgacttccgactaaaggtcttgccacattcattacacttgtaaagtttctctccagtatgaattatcctatgtctttcaaggtttgatttgaaactgaaagcttcatcacattcttcacatttgtaaggtttctctccagtatgaagtctacgatggtatacaagggatgatgtctgactgaaggtcttgccacaatcattacacttgtaaggtttctctccagtatgaattctcctatgtctttcaaggttcgatttgaaactgaaagcttcatcacattcttcacatttgtaaggtttctctccagtatgaagtctacgatggtatacaagggatgacatctgactgaaggtcttgccacaatcattacacttataaggtttctctccagtatgaagtctacgatggcgtgtaagggatgacttccgactaaaggtcctgctgcattcattacacttgtaaggtttctctccagtatgaattttcctatgtctttcaaggtttgatttgaaactgaaagctttgtcacattcttcacatttgtaaggtttctctccagtatgaagtctacgatggtacacaaggtatgacgtttgactgaaggtcttgccacattcattacacttgtaagatttctctccagtatgaattgccttatgaattacaagggctgaatttcgactgaaggtcttgccacactcactgcacttgtaatgtttctctccagtatgaagtctatgatggcatgtaagggttaactcctgactgaaggtcttgccacaatcattacacttgtaaggtttcttgccagtgtgacatctacgatgacatgcaagatatcgcttttgattaaagaccttgccacacacatcacatttatattgtttcgctcctaaatggattatctgatgtttccttaagactgagctataattaaaggctttgccactctcattacattggaaagatttttctctcatgtgtacttcctgcttttgtgtgagtaatgaagaattcaggaaattattcccatagttcttagaaatgtgggttttaggcctacaagaaattctttgggatgttgaaaccaacgaagcactgttgatagacttctcaacttgattaccaattttcccttcggtctgaaacatgtggagttcaggcagatgcgaatgaaagcttgatccaagctgatctttaataggcttgtttccagcatgcctttgatcatgtcggtttgtactacccgtcaactgtttgatttctgtcatgggtgcttcatggctatttctttcatcttctttccactgaaactcaaaatcatgaatatctttctccatttcctggaagcaaaaatctccaatgtgatgacgttcatgtctttgcaatgtccctgtgtggatcacttctgtattgccttgtgctgttgatgagaactccttcatcatgcatttggaagagatatccagggagaccaggttcctataattctccagcatcacgtccctgtatagagtcctctgagcagggtccaggcacttccactcttcctgagagaattctatggccacatccctgaatgtcaatagaccctgagaaagagccatccctgactcctttgctttcctcttcctcttccgggtttcttcctcacgtaccaagagtctttagaagtcaatcctgcagctgaggggccagcgagttccagcagagggacagcccacatgaacgccttgaggcaggagcaacctcggcccaggaacaggaaagacgcctgcatggcgctgcggtgggaccatcactccatgcgatccgcttccgggttt

SEQ ID NO: 11498 - RNA, 6420 nt, Homo sapiens
  source 1..6420: mol_type = other RNA
ctgaatagctgggactacaggtgcctgccacctcgcccagctaattttttgtatttttagtagagacggggtttcaccgtgttagccaggatggtctcgatctcctgacctcgtgatccgcccaccttagcctcccaaagtgctgggattacaggcgtgagccaccacgcccggcctcatttacaaattttctaaataaacgtcctgagaaaagagacaaaaggaagggaaatcttttcctttattctcaaaggaggaattatgcctctcatttatttgcttgtttgagacagggtctagctctgtcacccaggctggagtgcagtggtgagatcagggctcacttcagcctcaaaatccctgcttcaactgatcctcccacttcagtgcccagagtagctgggaccacagcagtgcaccaccacacctggctgactttttttacttttagcagagaagaggtcccctatgtcgcccaggctggtcttgaatccctaggctcacgtcacccacctgcctgggcctctaaaaccgctgggattacaggcctgagccactgcgtctggtctcatcgtaaatttgatgtttcttcttgttttaacagaatttgtattgctgtgatagaggttcttttcaaactgatgtcttatccttctgagtgcctcaaactagagcctgttcagacgttataacaagtttatactggtttattttggtacaaaaagtgtgaaatttatgcacaaatttttcataatatgtatttttccatgaacttcttgaagacccttatactagcaaactgtattcaagaggatataaaaagggattgtaaacatccaagtgctacctattcatgggatgcaaggatggttcaacatactcaaatcaatgggatacacacttgcacagaatgacagataaaaaacacattatctcaatagatagagaaaaagcatttcacagaactcaatattcattcttcgtaaaaatcctaaacaatataggtagagttttacctcaaaaatataaaaatcatccatgaaatgaccacagctgaaataaccaatgaaggaaaatggaatggttttcctgtaggatatcacatgatgcaagaatgctctcacccctgatattcaataaatactggctgtcctaggcagagcaattaaatagcaaaagaaataaaactcatccaaatcagaaagacagaagtaaaattacatttgttggggccgggctcatggctcacacccataatcccagcaatttgcaagtccgaagtgggcggataatgaggttaggcgatctaacatattctttcaagttctcttcaaggtactcaccatgttggcccaccatctgggccaacatggtgaaaccccgtctttactaaaataaaaaaaataaataaattagctaggtgtggtgacatgcgcctgtagtcccagctactcaggaggctgagacagaattgcttggacgtgggagacagaggttgcagtgagcaaagatcattccacggcactctagcctggcgacagagagagacattgtctcaaaaaaaaaaattatttccttgtagatgatacgacattctatatagaaaatcactggctgggtgcggtggctcacacctgtaatcccagaactttgggatgctgatgggggcggatcacctgaagtcaggagttcaagaaaaacctggtcaacatggtgaaaccccgtctctactaaaaatacaaaaaaattatacggacatggtggcaggcacctgtaatctcagttagtaggcaggagaatcacttaaacccgaaaggcagaggctgcagtgagccaagatcgtgccattgtactccagtccaagtgacaagagtgagactccttctcaaaaaaaaagaaaagagcctgggtaacagagtgagactgtctcaaaaaaaaaagaaagaaaatcacaaagaatcaaccaagattttactgatactaataaacccactcaatgtatttgcagaatacaaaatcagcacccaaaattagttgaatttccttacattaacaataaataatgtttaaagaaacttatgaacacacttcaatttgctatgaaacttaatacttacaaataaactgaattaaggaggtgagaagcttgtaccttgaaatctacattgatcaaaaaaactaaatagacatacaacccatattgatggattggaagtcttaatattgttgaatgattatacaaacaaatgtgatttagattcaacagatacccataaaaacccgtaacagtttttattaaagaaacaaaatacagggtgggaaaagtgactcatgtctgttggccagtctggtctcaaactcctgacctcaagtgatctattggtcttggcctcccaaagtgctgggattacaggcgtgagccaccccgcctggcccaatcttcttaacataaacactttaatgtcaattaatgcttgaactcaatgttaagtcaattcaaactcaagtcaatgctgaattgactctaatgccaattaatgcttgatggtttgctatactcattgcatttggaacaatcatctcaaaaatgaattttctgatgttccttaaggggtgatctcagactgaagaccttgccacactgatgacatttgtaagatttctgtccagtatggattctctgatgtctaattaggtgtgaacgtgaagtaaaggctttgctgcaatcatcatacttgtgaagtttgtctcctgtatgaagtctcctgttttgcataagatgaagctagactgaagaccttgccacaatcatgacatttgtaaggtttctctccagcatgagttcaccgatgaactgcaaggtatgaacaatgtctgaaaaatttgccacatttattacactttcaaaatctctcattatggattctccaatgatttgaaacggttgtagtgttactgaagactttgtgataatcattacattagtaaagtttccctataccatggattgcctgatggtgaataagtgttgactgcccactaaaggctttgccacactcagtacacttgtaaggtttctctccagtgtgacttctagtttgttgggccaggtgtgaatcacgcccaagattcttgtcacaaactcttacatttgtaagctttctctccagtatgaattctcctgtctttcaagacttgatttacaactgtaaactttgtcacattcttcatatttctaatgtttctttccagtatgaattctatgatgacgtgcaagttttgcttttcgattaaaaaccttgccacattcattacacttgtaaggtttctctccagtatgaattgtcttatgaattacaaggactgaattgtgacggaaggttttgccacactcattacacttgtaaggtttctctccagtatgaattctatgatgacatgcaaggtgtgcttgttgattaaaaaccttaccacatttattacacttgtaaggtttctctccagtatgaagtctatgatgacgtgaaaggtttgcttttctattaaaaaccttgccacattcactacacttgtaaggtttttctccagtatgaattgccttatgaatttcaagggctgaattgtgacggaaggtcttgccacactcattacacttgtaaggtttctctccactatgaattgccttatgaattacaagggctgaattgtgacggaagttcttgccacattcattacacttgtaaggtttctctccagtgtgaattctagtatgttgtgccaggtgtgaatcacgcccaaaagctttgtcacaaaccttacatttgtatggtttctctccagtatgaattctcctgtgtttttcaaggcttgatttgcgactgaaaactttgtcacattcttcacatttgtaaggtttctctccagtatgaagtctaagatggcatgtaagggatgacttctgactgaaggccttgccacactcattacacttgtaaggtttctctccagtatgaattgccttgtgaattataagggctgaatttcgaccgaaggtcttgccacactcattacacttgtaaggtttctctccagtatgaagtctacgatggcatgtaaggtatgacttccgactaaaggtcttgccacattcattacacctgtaaggtttctctccagtatgaattctcctatgtctttgaaggtttgatttgaaactgaaagcttcatcacattcttcacatttgtaaggtttctctccactatgagttcgccaatgaactgcaaggtatgaacgatgtctgaaaaatttgccacatctattacacttgtacgatctctcttcattatggattctccaatgatttgcaatggttgtagcattactaaagacttggtgacaatcattacatttgtaaagtttccctataccatggattgcttgatggtaaataagtgctgactgcccacgaaaggctttgccacactcattacactggtaaggtttctctccagtatgaagtctacaatggcgtgtaagggatgacttccgactaaaggtcttgccacattcattacacttgtaaagtttctctccagtatgaattatcctatgtctttcaaggtttgatttgaaactgaaagcttcatcacattcttcacatttgtaaggtttctctccagtatgaagtctacgatggtatacaagggatgatgtctgactgaaggtcttgccacaatcattacacttgtaaggtttctctccagtatgaattctcctatgtctttcaaggttcgatttgaaactgaaagcttcatcacattcttcacatttgtaaggtttctctccagtatgaagtctacgatggtatacaagggatgacatctgactgaaggtcttgccacaatcattacacttataaggtttctctccagtatgaagtctacgatggcgtgtaagggatgacttccgactaaaggtcctgctgcattcattacacttgtaaggtttctctccagtatgaattttcctatgtctttcaaggtttgatttgaaactgaaagctttgtcacattcttcacatttgtaaggtttctctccagtatgaagtctacgatggtacacaaggtatgacgtttgactgaaggtcttgccacattcattacacttgtaagatttctctccagtatgaattgccttatgaattacaagggctgaatttcgactgaaggtcttgccacactcactgcacttgtaatgtttctctccagtatgaagtctatgatggcatgtaagggttaactcctgactgaaggtcttgccacaatcattacacttgtaaggtttcttgccagtgtgacatctacgatgacatgcaagatatcgcttttgattaaagaccttgccacacacatcacatttatattgtttcgctcctaaatggattatctgatgtttccttaagactgagctataattaaaggctttgccactctcattacattggaaagatttttctctcatgtgtacttcctgcttttgtgtgagtaatgaagaattcaggaaattattcccatagttcttagaaatgtgggttttaggcctacaagaaattctttgggatgttgaaaccaacgaagcactgttgatagacttctcaacttgattaccaattttcccttcggtctgaaacatgtggagttcaggcagatgcgaatgaaagcttgatccaagctgatctttaataggcttgtttccagcatgcctttgatcatgtcggtttgtactacccgtcaactgtttgatttctgtcatgggtgcttcatggctatttctttcatcttctttccactgaaactcaaaatcatgaatatctttctccatttcctggaagcaaaaatctccaatgtgatgacgttcatgtctttgcaatgtccctgtgtggatcacttctgtattgccttgtgctgttgatgagaactccttcatcatgcatttggaagagatatccagggagaccaggttcctataattctccagcatcacgtccctgtatagagtcctctgagcagggtccaggcacttccactcttcctgagagaattctatggccacatccctgaatgtcaatagaccctgagaaagagccatccctgactcctttgctttcctcttcctcttccgggtttcttcctcacgtaccaagagtctttagaagtcaatcctgcagctgaggggccagcgagttccagcagagggacagcccacatgaacgccttgaggcaggagcaacctcggcccaggaacaggaaagacgcctgcatggctggagcagagggagggaggaggacacgggaaacagatgaggtcagagaggaccgctgcggtgggaccatcactccatgcgatccgcttccgggttt
